European Patent Application EP 4 520 821 A1 - sequence listing, part 2

SEQ ID NO: 8808 - RNA, 7726 nt, Homo sapiens
  source 1..7726: mol_type = other RNA
aagtgtgcagggcactggtgctgctccgaagctcatgaatacctttgctgcctagcacctctgtgccttgggcttcaaggccagggaagctgcacgctgatctcacaagagacactatctttttgaccagcagcttgccctccgcaatctgctgtcttagggcactgtagtcatcaatgtggccaatgacatggcggccatgcttattggcaaaggagccatcagtagcatcaccctctagcttgggaggggtcttcattactggagaagtatccaaacccaagccatttgctctgttgattatgggcgtttctgagccaggagtagaggaagcagagctggggaagaccagagctggggaattcataccaacatcccggactggaggggacacagctgaatcttggaggagcagctgcttgtttccagggtcagtgctggctgggaagttctggttaatggaggaggggctgaggctggctttgccagcaccgctctccagctgctgttgcagctgcagtcgcagacaattgttcccctgaatgctctgctccagctgccctctcagagctcgtacctctgccaccaggtggctcaggtcactgctcaaagggatttggtgacaggcatccaggctgtaagctttcagccccttcttggaattgccataaagtgcctcgtagatttgtagctctgactggagggactcaaagagctgctgtttctcttcacactgttgctgcaggagaaccagcttgtgctgcagtctggagtcgttttcctggagggaaagacgttcctccctgaaatgcaagacctcttgctgcttctccctcaagtcttccaaaagctgctgcctttccaccttctggtgctccagctccttttccagctcttgaaggtgggatcgagaggacagcagagcctccctcaggctttctgtttcctgggagtgctctctggaaacatgactcagttgagcctgaagtcttcgattgtcttccctgaggactctgttctcattgcagagctgaggtatggactccaggccctgactgtagaagttagaagtggatccccttccacgagcagtagaggtcagccggtgttccagttgctcccgtaggcggtcattgatgcagatggattcctccaggcgctggcgcaggttccggatttcaccaagatgctcttccagcaggtcagcccctgtgggtttggagttaagctggtacacagaggagcctgaggataggtccccagatacactccctttctgaggcctcatcacatcccacttgccactgctgcccaggtacccaggctctaggattcttcccagttctatggtgccccttggaggagagtgaggctgggcagagttgaggtagtaggaagagtcggcttccaagtcgttgctcagcaatgtagctgtggaagcaggaggaacagtgctggcactttctcccaactgcttctgcagcatctgtagctcctgctgagcctcagccaaggagaccactggtgtctcacagcagccaaggaggagagggccagtggggctgaaaggcaggaagctggatggagctgagggcaatggtgcctgaggaaggctagccagcttgggtatggagtgaaaatgaaagcctgaatgggcctggttggcctccttgggggtattctggggagttggcaagctgatggggttgctgttggattcggccttagccccctgagatgcactggttgatgatggtttagaagacaacacagcagaatgactcgaatgatggatggaatctgagtgactgggagaagctttcttctcttcatagtgtgtgtactcgctgactatgtccatgtcagagcaggcttccagttcatcagacaggaaagaggtgctgctgggagagcggtgggagtcagacaaggcatggctgctggagggtgtgagggaccgagcatccagcttggcctgcaggacttcaatcactttctccttctcctgcagctccctgctgagcctgagggccagtggctcaagtccagcttgatctttctcacttttatgatccttggtgctgagtttgctggtgagcctctctgtcagctggcttccctgggcgagttgctcccggaagctctgtcccaggtagtagtcaatgtcattgctccttaggagatcctcaaaagattttactgtatcttttgcatgccgggtgataagataacaaatacctctcccttctcgtattttttgccgtaggtaagacagttcccgggcctgatcctgaatcagggaatcatatttcccaggccacgaggctgatctcagctcctcagccagcttctcttctagtccattttttgggagctgggcctccagctgggatactctctggatgagactctccaggtcctttttggcctgaagccctggagagtagaaagccccagtgccatcagacagccacccctcatcctcatcagggacactatgaggtgaagacccctccaaggtgccaacagctctcagcttccggggtctttccagactagacgaataatcacttgtaactgagagggaccggacccggctcttgaggttttgaatgaccttgttggcattctgcagctgggccttcagatctttgatgtcctttcgtaggaccaagatgttttctgactttccatatacccggaactcttcctgcttccctagctggttctccaagggcttcctctcagaggaactagccagtgttgagccccggcgtccctgctcagagcacagcccctccatcaggaccatttccttgaggctgttgtgctcctcacactcaggactggtggtttcctcccgttcagcctcattctcgcttcggccacaagtctcatagcccaggtcctggaggtccacctggatctgcttgctgtcctgcttcaccaaggattcacctgtaagcataactctgtatttctccagctcgttagcctgagcaaagacagtggcttctgatagcagcagcttctcctggagatcttgatagcgttgtttgcattgtgacagctgggagcgcaggtgctgggtggaccctggtaggctaaacgctgactgaggcccagggtcacgaggctgggactggttatccaattggtgggcatccactgtgaaggtagccccaaggtcaaggctctggggtctggggaaaggcctcacagtcacattcccctcctcttggtgttggtgcttcccaggggaaccaaccagttctgtgtttattctttcaatggtgctggtcagatgcacaaggagctctggagtaagtttactattcccttccttgctactcagcacaagttgttctttgaggaggttgatgatattgtgggcattcttcagttttccctggagctttctgaactcagcctgaaggctactctcactcagaccctctttggttaccacagtctcaaccatcacctcgcccttctccttgtcttcctcgatctcccatccatcagacattgcttctcccatctgctctttcagctccgcattctcaaggcaaaggctcagcatggtgttcctgatgtgggacactgaggagaatcctgcttcctcaatttgagcctttagctccttcagttcctcctcagctttcctcttctcttctaagtgctggtggaactcagccctcaggtggagcatttcttcctgaagacacctgttactgtcccctcccatcggagaaggaggggaaaaagatgggttctgggtctccacagttgccagacttttctccaaagccaccttgacaagttgctggtgactatggtgtgcagcctcctcctcaatactgtcagtgaactcagtgcttgtatcttcggtgtcatcccctgcagctgcacctccaatggcggccagggtctccagcctgtttaagcgctccaagcttcttccaagaacttcttctagccgactgcgtaacacctgagccccttccagttccacctgcagagttcggtctctctcagagctctctggatgggcatggaacttcaccagactgctatagagctgtctctctgcttgtaaggcctcattgagccgactccgttcatctactagtccttctagcatcagcagcaactgttgtcttcggtttcctgaaatttcttgaccctgggattctactgaagcaactttttcccgaagaagtaagacttcctgggtcaggcgttccatagctggtatgtcttcaggatcaaccagttgcatttgcaggtcctttatgagatcttctttaatctgtatgttcctggtcagagactccatatcagcagcctgcacctgcagctcttcttcctgcacagccatcatggactgtagagcagaaagttccatctgactttctctttcttttttagccatgagttcaagttcctctttggcattactcagttctttttccagccctgcaactgtgtccaagtctcctaatgtggatctgggtatgctgacatcctctttggcagtcaatgaagtgctatcatctctggaaggtatctgcattgaaccttgatcagtctgttttccaagacggccagtgggggtaacttcagcttgttggttagagatgggtgcttgggacatcagggagtctctccctcctaaatattggcgcagggcctgtaattctgaatttctttccattaaggcttgcaccaacttctctgcagcagcttggctttcctgctccctggtgctcacagactgaagcaggccttgaatctccatttcatgttccagcacttgtttatttcgatcacttagaaggtcctgcagcatcctttcctttcgctgtagacgctggcacagctcctctgctatctcactctgccctggtccaagtttgcagagcagtgttgcactaagatcctccacttctttgttcctatcatgaagagacgtctgtaactgctgaatgatactctcttgttccttctgccaacggctaaatttggtttccatttcttctttcagccactggaggttttgacaggtagtagataactgttccacttccaggcctttggccctcaggagactctccatactttgcatagtagcttcattggaggagaggacatcgcgcagtctctctaagtcatgatctcgctctctcacagcaagacgaagctggcgcagttctttttctttctcttctagagcagagaatttttcatctatagcccgctccagagcaacagctttatcatgtattcgctggcgaagtttctcaagcaacatttcatttgcttcaagggttttgtctgagttatctcgatactgtaggagctcccgaaattcctgaagcaactgctccttgtgactcagactatggtttaggtgctggatgttttgttcctgggttcgaatctcattgtatttttcagcctcccaggcacgaagctgttggctcttattctgcaattcttcttgtagctgctgcaaggcttttcgcaattcctggttatgtttccaagaagcctctttctgctgttcactctcgtgtgctgcagcctctacaaattgcacacattgtttggcatcagccagttggcgctctttctgtcgtaccaccctctggagcttctgtatttcaagttggctgcagaataaagcactctgaagatcaagcagagctacctgttgctgagctggagaagtaccctctgagctgtgaagttgtccaagctggctttggtgcagcatttctcgaagctttgccattgtgtcattttgaccttcaattacctggtacaactcctcagtctcacgttccctgcttttcagagtttccttgaggttctgaattgtaccatcttgcttttgagacgactcctgagcacactttagttcatagctcatttcattaagtttctcttgaagaatcttgttggtggcctctgtttgctggattttttcctggagttctgccaagtgggaatcagatacagactgctgagttatagtggtctcatgtgaattcagcttttgttgtttcagcaactcttcagtcatgggctgcacttccatgctagttggctcctccaacagatgtagcagttgttgtttctcccgagatagctgttctacaagcctctcctgggcagccaggctctgattcagttcttcaattctcttgtccctctgggccagggcctcagtgtattggtcgggcttgacctggtctcctggtacatcttcccagtttttggtgactcccttcagtttctctgagagctccaggttacactccttctctgcttccaccagagctgccatccgcgcagcttcattctttgctagcctggattcctcctgcagaagctggatcttattctccaagagctcataaacatgctccgtctcctgctgtcgctcctcaaactggcgtcggagctcagcttcattctgactgttgagattctccacatcagcccatgttttatccagatgctgtttcttgtcctggagttctcgtttcaagctctccacttcaaccttcagctcaatgttccgcttgtagatgtcctcccggctggcctcatacttctgttgcatgcgctcctccaggaagtagatgcgcagcttgaggctgaagttctccttcttcaggtcattgaggtgcttctcaaagtctcgaagagcctgggtctgtacctgagggggtttctcaaatgctctcaaggaatatgtctgcacaaacgggaccttttcaccacttctccagatctgtgactgcactggagggcctcgatctttagtgtcactaagaaaagcagaaggagcccaagaaaaagcacccagatgcttcagtcaacttcttagaattcttcttttttttatgttcagaaaagatggaaattcatttctgctgtgtgactcgttctgggtaccatctccccatcatcctctgcaaaataatctctcgtccaggtctgctccattttccaggctctttccttagtctcaggacgctcctcacccgggaggggaagcagcctgggaaaatgagaagccttgcccacgaatctccagcgcaaaaggcagcagctttttcctccccagctcctttctgcgtcggcggcgaagagagagctctgctccctgcttttttagaaaatggatttgacgtggccgaacctgcggctagccgtgcgacccgcacaagggagggactgttctcagtaggaggctggactcagagcggcgcggcgcccggggctgtttcgtgagctggagccagcggctgcccgggccgcggtgcgcgcactctccaggctgagacacgactggctggcacgagttgctcggcaccagctgagctgtcaaccgcgagcggaggcggggctcccgacaaccagtgtgctggggcagaatcggcccaggttacacgccccctgaaccaccctcgcgtctccccgacccctctctcgctggctcagatgaatgatgacggcagagggcagagagcttagaggacgcggtaccaagccccgtccctcgcccatcccaacgaaggtcttagaatacaatcaaccaactacaggaagaatttgtagaggaggttttcttgtgtgtctgcatcgccccacccacaggtaaccccagagccagagatggagtctaggaaggtttaggagcaatcccggctga

SEQ ID NO: 8809 - RNA, 7301 nt, Homo sapiens
  source 1..7301: mol_type = other RNA
aagtgtgcagggcactggtgctgctccgaagctcatgaatacctttgctgcctagcacctctgtgccttgggcttcaaggccagggaagctgcacgctgatctcacaagagacactatctttttgaccagcagcttgccctccgcaatctgctgtcttagggcactgtagtcatcaatgtggccaatgacatggcggccatgcttattggcaaaggagccatcagtagcatcaccctctagcttgggaggggtcttcattactggagaagtatccaaacccaagccatttgctctgttgattatgggcgtttctgagccaggagtagaggaagcagagctggggaagaccagagctggggaattcataccaacatcccggactggaggggacacagctgaatcttggaggagcagctgcttgtttccagggtcagtgctggctgggaagttctggttaatggaggaggggctgaggctggctttgccagcaccgctctccagctgctgttgcagctgcagtcgcagacaattgttcccctgaatgctctgctccagctgccctctcagagctcgtacctctgccaccaggtggctcaggtcactgctcaaagggatttggtgacaggcatccaggctgtaagctttcagccccttcttggaattgccataaagtgcctcgtagatttgtagctctgactggagggactcaaagagctgctgtttctcttcacactgttgctgcaggagaaccagcttgtgctgcagtctggagtcgttttcctggagggaaagacgttcctccctgaaatgcaagacctcttgctgcttctccctcaagtcttccaaaagctgctgcctttccaccttctggtgctccagctccttttccagctcttgaaggtgggatcgagaggacagcagagcctccctcaggctttctgtttcctgggagtgctctctggaaacatgactcagttgagcctgaagtcttcgattgtcttccctgaggactctgttctcattgcagagctgaggtatggactccaggccctgactgtagaagttagaagtggatccccttccacgagcagtagaggtcagccggtgttccagttgctcccgtaggcggtcattgatgcagatggattcctccaggcgctggcgcaggttccggatttcaccaagatgctcttccagcaggtcagcccctgtgggtttggagttaagctggtacacagaggagcctgaggataggtccccagatacactccctttctgaggcctcatcacatcccacttgccactgctgcccaggtacccaggctctaggattcttcccagttctatggtgccccttggaggagagtgaggctgggcagagttgaggtagtaggaagagtcggcttccaagtcgttgctcagcaatgtagctgtggaagcaggaggaacagtgctggcactttctcccaactgcttctgcagcatctgtagctcctgctgagcctcagccaaggagaccactggtgtctcacagcagccaaggaggagagggccagtggggctgaaaggcaggaagctggatggagctgagggcaatggtgcctgaggaaggctagccagcttgggtatggagtgaaaatgaaagcctgaatgggcctggttggcctccttgggggtattctggggagttggcaagctgatggggttgctgttggattcggccttagccccctgagatgcactggttgatgatggtttagaagacaacacagcagaatgactcgaatgatggatggaatctgagtgactgggagaagctttcttctcttcatagtgtgtgtactcgctgactatgtccatgtcagagcaggcttccagttcatcagacaggaaagaggtgctgctgggagagcggtgggagtcagacaaggcatggctgctggagggtgtgagggaccgagcatccagcttggcctgcaggacttcaatcactttctccttctcctgcagctccctgctgagcctgagggccagtggctcaagtccagcttgatctttctcacttttatgatccttggtgctgagtttgctggtgagcctctctgtcagctggcttccctgggcgagttgctcccggaagctctgtcccaggtagtagtcaatgtcattgctccttaggagatcctcaaaagattttactgtatcttttgcatgccgggtgataagataacaaatacctctcccttctcgtattttttgccgtaggtaagacagttcccgggcctgatcctgaatcagggaatcatatttcccaggccacgaggctgatctcagctcctcagccagcttctcttctagtccattttttgggagctgggcctccagctgggatactctctggatgagactctccaggtcctttttggcctgaagccctggagagtagaaagccccagtgccatcagacagccacccctcatcctcatcagggacactatgaggtgaagacccctccaaggtgccaacagctctcagcttccggggtctttccagactagacgaataatcacttgtaactgagagggaccggacccggctcttgaggttttgaatgaccttgttggcattctgcagctgggccttcagatctttgatgtcctttcgtaggaccaagatgttttctgactttccatatacccggaactcttcctgcttccctagctggttctccaagggcttcctctcagaggaactagccagtgttgagccccggcgtccctgctcagagcacagcccctccatcaggaccatttccttgaggctgttgtgctcctcacactcaggactggtggtttcctcccgttcagcctcattctcgcttcggccacaagtctcatagcccaggtcctggaggtccacctggatctgcttgctgtcctgcttcaccaaggattcacctgtaagcataactctgtatttctccagctcgttagcctgagcaaagacagtggcttctgatagcagcagcttctcctggagatcttgatagcgttgtttgcattgtgacagctgggagcgcaggtgctgggtggaccctggtaggctaaacgctgactgaggcccagggtcacgaggctgggactggttatccaattggtgggcatccactgtgaaggtagccccaaggtcaaggctctggggtctggggaaaggcctcacagtcacattcccctcctcttggtgttggtgcttcccaggggaaccaaccagttctgtgtttattctttcaatggtgctggtcagatgcacaaggagctctggagtaagtttactattcccttccttgctactcagcacaagttgttctttgaggaggttgatgatattgtgggcattcttcagttttccctggagctttctgaactcagcctgaaggctactctcactcagaccctctttggttaccacagtctcaaccatcacctcgcccttctccttgtcttcctcgatctcccatccatcagacattgcttctcccatctgctctttcagctccgcattctcaaggcaaaggctcagcatggtgttcctgatgtgggacactgaggagaatcctgcttcctcaatttgagcctttagctccttcagttcctcctcagctttcctcttctcttctaagtgctggtggaactcagccctcaggtggagcatttcttcctgaagacacctgttactgtcccctcccatcggagaaggaggggaaaaagatgggttctgggtctccacagttgccagacttttctccaaagccaccttgacaagttgctggtgactatggtgtgcagcctcctcctcaatactgtcagtgaactcagtgcttgtatcttcggtgtcatcccctgcagctgcacctccaatggcggccagggtctccagcctgtttaagcgctccaagcttcttccaagaacttcttctagccgactgcgtaacacctgagccccttccagttccacctgcagagttcggtctctctcagagctctctggatgggcatggaacttcaccagactgctatagagctgtctctctgcttgtaaggcctcattgagccgactccgttcatctactagtccttctagcatcagcagcaactgttgtcttcggtttcctgaaatttcttgaccctgggattctactgaagcaactttttcccgaagaagtaagacttcctgggtcaggcgttccatagctggtatgtcttcaggatcaaccagttgcatttgcaggtcctttatgagatcttctttaatctgtatgttcctggtcagagactccatatcagcagcctgcacctgcagctcttcttcctgcacagccatcatggactgtagagcagaaagttccatctgactttctctttcttttttagccatgagttcaagttcctctttggcattactcagttctttttccagccctgcaactgtgtccaagtctcctaatgtggatctgggtatgctgacatcctctttggcagtcaatgaagtgctatcatctctggaaggtatctgcattgaaccttgatcagtctgttttccaagacggccagtgggggtaacttcagcttgttggttagagatgggtgcttgggacatcagggagtctctccctcctaaatattggcgcagggcctgtaattctgaatttctttccattaaggcttgcaccaacttctctgcagcagcttggctttcctgctccctggtgctcacagactgaagcaggccttgaatctccatttcatgttccagcacttgtttatttcgatcacttagaaggtcctgcagcatcctttcctttcgctgtagacgctggcacagctcctctgctatctcactctgccctggtccaagtttgcagagcagtgttgcactaagatcctccacttctttgttcctatcatgaagagacgtctgtaactgctgaatgatactctcttgttccttctgccaacggctaaatttggtttccatttcttctttcagccactggaggttttgacaggtagtagataactgttccacttccaggcctttggccctcaggagactctccatactttgcatagtagcttcattggaggagaggacatcgcgcagtctctctaagtcatgatctcgctctctcacagcaagacgaagctggcgcagttctttttctttctcttctagagcagagaatttttcatctatagcccgctccagagcaacagctttatcatgtattcgctggcgaagtttctcaagcaacatttcatttgcttcaagggttttgtctgagttatctcgatactgtaggagctcccgaaattcctgaagcaactgctccttgtgactcagactatggtttaggtgctggatgttttgttcctgggttcgaatctcattgtatttttcagcctcccaggcacgaagctgttggctcttattctgcaattcttcttgtagctgctgcaaggcttttcgcaattcctggttatgtttccaagaagcctctttctgctgttcactctcgtgtgctgcagcctctacaaattgcacacattgtttggcatcagccagttggcgctctttctgtcgtaccaccctctggagcttctgtatttcaagttggctgcagaataaagcactctgaagatcaagcagagctacctgttgctgagctggagaagtaccctctgagctgtgaagttgtccaagctggctttggtgcagcatttctcgaagctttgccattgtgtcattttgaccttcaattacctggtacaactcctcagtctcacgttccctgcttttcagagtttccttgaggttctgaattgtaccatcttgcttttgagacgactcctgagcacactttagttcatagctcatttcattaagtttctcttgaagaatcttgttggtggcctctgtttgctggattttttcctggagttctgccaagtgggaatcagatacagactgctgagttatagtggtctcatgtgaattcagcttttgttgtttcagcaactcttcagtcatgggctgcacttccatgctagttggctcctccaacagatgtagcagttgttgtttctcccgagatagctgttctacaagcctctcctgggcagccaggctctgattcagttcttcaattctcttgtccctctgggccagggcctcagtgtattggtcgggcttgacctggtctcctggtacatcttcccagtttttggtgactcccttcagtttctctgagagctccaggttacactccttctctgcttccaccagagctgccatccgcgcagcttcattctttgctagcctggattcctcctgcagaagctggatcttattctccaagagctcataaacatgctccgtctcctgctgtcgctcctcaaactggcgtcggagctcagcttcattctgactgttgagattctccacatcagcccatgttttatccagatgctgtttcttgtcctggagttctcgtttcaagctctccacttcaaccttcagctcaatgttccgcttgtagatgtcctcccggctggcctcatacttctgttgcatgcgctcctccaggaagtagatgcgcagcttgaggctgaagttctccttcttcaggtcattgaggtgcttctcaaagtctcgaagagcctgggtctgtacctgagggggtttctcaaatgctctcaaggaatatgtctgcacaaacgggaccttttcaccacttctccagatctgtgactgcactggagggcctcgatctttagtgtcactaagaaaagctgctgtgtgactcgttctgggtaccatctccccatcatcctctgcaaaataatctctcatccagggtgtggccgccgcagctgcttcttcctcctcggccgctgctgcccagctcccggctggctccgggcgccgtctttcccggctcggggtctgccgtggggactgaggggttcgcgtcgcgtccccggaccggtaaggcgtgtagtgagcccggcgggacgcgcgacagcagcagccaaagtcgcatcggcggcggcagcaggacccgctgtctgtgcccttcatggatttcctgggcctggccaccccagtcctagctacggttcctgcttgttttcctggtgttttccgggactgccagggcgcatcctctgggcctggctgagcatccccgtcagttccctgggcctcctccgcggctgcctctgccacctgctccgcccagatt

SEQ ID NO: 8810 - RNA, 7445 nt, Homo sapiens
  source 1..7445: mol_type = other RNA
aagtgtgcagggcactggtgctgctccgaagctcatgaatacctttgctgcctagcacctctgtgccttgggcttcaaggccagggaagctgcacgctgatctcacaagagacactatctttttgaccagcagcttgccctccgcaatctgctgtcttagggcactgtagtcatcaatgtggccaatgacatggcggccatgcttattggcaaaggagccatcagtagcatcaccctctagcttgggaggggtcttcattactggagaagtatccaaacccaagccatttgctctgttgattatgggcgtttctgagccaggagtagaggaagcagagctggggaagaccagagctggggaattcataccaacatcccggactggaggggacacagctgaatcttggaggagcagctgcttgtttccagggtcagtgctggctgggaagttctggttaatggaggaggggctgaggctggctttgccagcaccgctctccagctgctgttgcagctgcagtcgcagacaattgttcccctgaatgctctgctccagctgccctctcagagctcgtacctctgccaccaggtggctcaggtcactgctcaaagggatttggtgacaggcatccaggctgtaagctttcagccccttcttggaattgccataaagtgcctcgtagatttgtagctctgactggagggactcaaagagctgctgtttctcttcacactgttgctgcaggagaaccagcttgtgctgcagtctggagtcgttttcctggagggaaagacgttcctccctgaaatgcaagacctcttgctgcttctccctcaagtcttccaaaagctgctgcctttccaccttctggtgctccagctccttttccagctcttgaaggtgggatcgagaggacagcagagcctccctcaggctttctgtttcctgggagtgctctctggaaacatgactcagttgagcctgaagtcttcgattgtcttccctgaggactctgttctcattgcagagctgaggtatggactccaggccctgactgtagaagttagaagtggatccccttccacgagcagtagaggtcagccggtgttccagttgctcccgtaggcggtcattgatgcagatggattcctccaggcgctggcgcaggttccggatttcaccaagatgctcttccagcaggtcagcccctgtgggtttggagttaagctggtacacagaggagcctgaggataggtccccagatacactccctttctgaggcctcatcacatcccacttgccactgctgcccaggtacccaggctctaggattcttcccagttctatggtgccccttggaggagagtgaggctgggcagagttgaggtagtaggaagagtcggcttccaagtcgttgctcagcaatgtagctgtggaagcaggaggaacagtgctggcactttctcccaactgcttctgcagcatctgtagctcctgctgagcctcagccaaggagaccactggtgtctcacagcagccaaggaggagagggccagtggggctgaaaggcaggaagctggatggagctgagggcaatggtgcctgaggaaggctagccagcttgggtatggagtgaaaatgaaagcctgaatgggcctggttggcctccttgggggtattctggggagttggcaagctgatggggttgctgttggattcggccttagccccctgagatgcactggttgatgatggtttagaagacaacacagcagaatgactcgaatgatggatggaatctgagtgactgggagaagctttcttctcttcatagtgtgtgtactcgctgactatgtccatgtcagagcaggcttccagttcatcagacaggaaagaggtgctgctgggagagcggtgggagtcagacaaggcatggctgctggagggtgtgagggaccgagcatccagcttggcctgcaggacttcaatcactttctccttctcctgcagctccctgctgagcctgagggccagtggctcaagtccagcttgatctttctcacttttatgatccttggtgctgagtttgctggtgagcctctctgtcagctggcttccctgggcgagttgctcccggaagctctgtcccaggtagtagtcaatgtcattgctccttaggagatcctcaaaagattttactgtatcttttgcatgccgggtgataagataacaaatacctctcccttctcgtattttttgccgtaggtaagacagttcccgggcctgatcctgaatcagggaatcatatttcccaggccacgaggctgatctcagctcctcagccagcttctcttctagtccattttttgggagctgggcctccagctgggatactctctggatgagactctccaggtcctttttggcctgaagccctggagagtagaaagccccagtgccatcagacagccacccctcatcctcatcagggacactatgaggtgaagacccctccaaggtgccaacagctctcagcttccggggtctttccagactagacgaataatcacttgtaactgagagggaccggacccggctcttgaggttttgaatgaccttgttggcattctgcagctgggccttcagatctttgatgtcctttcgtaggaccaagatgttttctgactttccatatacccggaactcttcctgcttccctagctggttctccaagggcttcctctcagaggaactagccagtgttgagccccggcgtccctgctcagagcacagcccctccatcaggaccatttccttgaggctgttgtgctcctcacactcaggactggtggtttcctcccgttcagcctcattctcgcttcggccacaagtctcatagcccaggtcctggaggtccacctggatctgcttgctgtcctgcttcaccaaggattcacctgtaagcataactctgtatttctccagctcgttagcctgagcaaagacagtggcttctgatagcagcagcttctcctggagatcttgatagcgttgtttgcattgtgacagctgggagcgcaggtgctgggtggaccctggtaggctaaacgctgactgaggcccagggtcacgaggctgggactggttatccaattggtgggcatccactgtgaaggtagccccaaggtcaaggctctggggtctggggaaaggcctcacagtcacattcccctcctcttggtgttggtgcttcccaggggaaccaaccagttctgtgtttattctttcaatggtgctggtcagatgcacaaggagctctggagtaagtttactattcccttccttgctactcagcacaagttgttctttgaggaggttgatgatattgtgggcattcttcagttttccctggagctttctgaactcagcctgaaggctactctcactcagaccctctttggttaccacagtctcaaccatcacctcgcccttctccttgtcttcctcgatctcccatccatcagacattgcttctcccatctgctctttcagctccgcattctcaaggcaaaggctcagcatggtgttcctgatgtgggacactgaggagaatcctgcttcctcaatttgagcctttagctccttcagttcctcctcagctttcctcttctcttctaagtgctggtggaactcagccctcaggtggagcatttcttcctgaagacacctgttactgtcccctcccatcggagaaggaggggaaaaagatgggttctgggtctccacagttgccagacttttctccaaagccaccttgacaagttgctggtgactatggtgtgcagcctcctcctcaatactgtcagtgaactcagtgcttgtatcttcggtgtcatcccctgcagctgcacctccaatggcggccagggtctccagcctgtttaagcgctccaagcttcttccaagaacttcttctagccgactgcgtaacacctgagccccttccagttccacctgcagagttcggtctctctcagagctctctggatgggcatggaacttcaccagactgctatagagctgtctctctgcttgtaaggcctcattgagccgactccgttcatctactagtccttctagcatcagcagcaactgttgtcttcggtttcctgaaatttcttgaccctgggattctactgaagcaactttttcccgaagaagtaagacttcctgggtcaggcgttccatagctggtatgtcttcaggatcaaccagttgcatttgcaggtcctttatgagatcttctttaatctgtatgttcctggtcagagactccatatcagcagcctgcacctgcagctcttcttcctgcacagccatcatggactgtagagcagaaagttccatctgactttctctttcttttttagccatgagttcaagttcctctttggcattactcagttctttttccagccctgcaactgtgtccaagtctcctaatgtggatctgggtatgctgacatcctctttggcagtcaatgaagtgctatcatctctggaaggtatctgcattgaaccttgatcagtctgttttccaagacggccagtgggggtaacttcagcttgttggttagagatgggtgcttgggacatcagggagtctctccctcctaaatattggcgcagggcctgtaattctgaatttctttccattaaggcttgcaccaacttctctgcagcagcttggctttcctgctccctggtgctcacagactgaagcaggccttgaatctccatttcatgttccagcacttgtttatttcgatcacttagaaggtcctgcagcatcctttcctttcgctgtagacgctggcacagctcctctgctatctcactctgccctggtccaagtttgcagagcagtgttgcactaagatcctccacttctttgttcctatcatgaagagacgtctgtaactgctgaatgatactctcttgttccttctgccaacggctaaatttggtttccatttcttctttcagccactggaggttttgacaggtagtagataactgttccacttccaggcctttggccctcaggagactctccatactttgcatagtagcttcattggaggagaggacatcgcgcagtctctctaagtcatgatctcgctctctcacagcaagacgaagctggcgcagttctttttctttctcttctagagcagagaatttttcatctatagcccgctccagagcaacagctttatcatgtattcgctggcgaagtttctcaagcaacatttcatttgcttcaagggttttgtctgagttatctcgatactgtaggagctcccgaaattcctgaagcaactgctccttgtgactcagactatggtttaggtgctggatgttttgttcctgggttcgaatctcattgtatttttcagcctcccaggcacgaagctgttggctcttattctgcaattcttcttgtagctgctgcaaggcttttcgcaattcctggttatgtttccaagaagcctctttctgctgttcactctcgtgtgctgcagcctctacaaattgcacacattgtttggcatcagccagttggcgctctttctgtcgtaccaccctctggagcttctgtatttcaagttggctgcagaataaagcactctgaagatcaagcagagctacctgttgctgagctggagaagtaccctctgagctgtgaagttgtccaagctggctttggtgcagcatttctcgaagctttgccattgtgtcattttgaccttcaattacctggtacaactcctcagtctcacgttccctgcttttcagagtttccttgaggttctgaattgtaccatcttgcttttgagacgactcctgagcacactttagttcatagctcatttcattaagtttctcttgaagaatcttgttggtggcctctgtttgctggattttttcctggagttctgccaagtgggaatcagatacagactgctgagttatagtggtctcatgtgaattcagcttttgttgtttcagcaactcttcagtcatgggctgcacttccatgctagttggctcctccaacagatgtagcagttgttgtttctcccgagatagctgttctacaagcctctcctgggcagccaggctctgattcagttcttcaattctcttgtccctctgggccagggcctcagtgtattggtcgggcttgacctggtctcctggtacatcttcccagtttttggtgactcccttcagtttctctgagagctccaggttacactccttctctgcttccaccagagctgccatccgcgcagcttcattctttgctagcctggattcctcctgcagaagctggatcttattctccaagagctcataaacatgctccgtctcctgctgtcgctcctcaaactggcgtcggagctcagcttcattctgactgttgagattctccacatcagcccatgttttatccagatgctgtttcttgtcctggagttctcgtttcaagctctccacttcaaccttcagctcaatgttccgcttgtagatgtcctcccggctggcctcatacttctgttgcatgcgctcctccaggaagtagatgcgcagcttgaggctgaagttctccttcttcaggtcattgaggtgcttctcaaagtctcgaagagcctgggtctgtacctgagggggtttctcaaatgctctcaaggaatatgtctgcacaaacgggaccttttcaccacttctccagatctgtgactgcactggagggcctcgatctttagtgtcactaagaaaagctgctgtgtgactcgttctgggtaccatctccccatcatcctctgcaaaataatctctcatccagggtgtggccgccgcagctgcttcttcctcctcggccgctgctgcccagctcccggctggctccgggcgccgtctttcccggctcggggtctgccgtggggactgaggggttcgcgtcgcgtccccggaccggtaaggcgtgtagtgagcccggcgggacgcgcgacagcagcagccaaagtcgcatcggcggcggcagcaggacccgctgtctgtgcccttcatggatttcctgggcctggccaccccagtcctagctacggttcctgcttgttttcctggtgttttccgggactgccagggcgcatcctctgggcctggctgagcatccccgtcagttccctgggcctcctccgcggctgcctctgccacctgctccgcccagattgctttggtccttctcccgcagacacactcagctgcccttcatcctctgtcgtctccccattctctctccacccactgcctcattcccagatcccacgccgtttcttcctttctatccgctccaatgtcaccttctctttatttc

SEQ ID NO: 8811 - RNA, 7273 nt, Homo sapiens
  source 1..7273: mol_type = other RNA
aagtgtgcagggcactggtgctgctccgaagctcatgaatacctttgctgcctagcacctctgtgccttgggcttcaaggccagggaagctgcacgctgatctcacaagagacactatctttttgaccagcagcttgccctccgcaatctgctgtcttagggcactgtagtcatcaatgtggccaatgacatggcggccatgcttattggcaaaggagccatcagtagcatcaccctctagcttgggaggggtcttcattactggagaagtatccaaacccaagccatttgctctgttgattatgggcgtttctgagccaggagtagaggaagcagagctggggaagaccagagctggggaattcataccaacatcccggactggaggggacacagctgaatcttggaggagcagctgcttgtttccagggtcagtgctggctgggaagttctggttaatggaggaggggctgaggctggctttgccagcaccgctctccagctgctgttgcagctgcagtcgcagacaattgttcccctgaatgctctgctccagctgccctctcagagctcgtacctctgccaccaggtggctcaggtcactgctcaaagggatttggtgacaggcatccaggctgtaagctttcagccccttcttggaattgccataaagtgcctcgtagatttgtagctctgactggagggactcaaagagctgctgtttctcttcacactgttgctgcaggagaaccagcttgtgctgcagtctggagtcgttttcctggagggaaagacgttcctccctgaaatgcaagacctcttgctgcttctccctcaagtcttccaaaagctgctgcctttccaccttctggtgctccagctccttttccagctcttgaaggtgggatcgagaggacagcagagcctccctcaggctttctgtttcctgggagtgctctctggaaacatgactcagttgagcctgaagtcttcgattgtcttccctgaggactctgttctcattgcagagctgaggtatggactccaggccctgactgtagaagttagaagtggatccccttccacgagcagtagaggtcagccggtgttccagttgctcccgtaggcggtcattgatgcagatggattcctccaggcgctggcgcaggttccggatttcaccaagatgctcttccagcaggtcagcccctgtgggtttggagttaagctggtacacagaggagcctgaggataggtccccagatacactccctttctgaggcctcatcacatcccacttgccactgctgcccaggtacccaggctctaggattcttcccagttctatggtgccccttggaggagagtgaggctgggcagagttgaggtagtaggaagagtcggcttccaagtcgttgctcagcaatgtagctgtggaagcaggaggaacagtgctggcactttctcccaactgcttctgcagcatctgtagctcctgctgagcctcagccaaggagaccactggtgtctcacagcagccaaggaggagagggccagtggggctgaaaggcaggaagctggatggagctgagggcaatggtgcctgaggaaggctagccagcttgggtatggagtgaaaatgaaagcctgaatgggcctggttggcctccttgggggtattctggggagttggcaagctgatggggttgctgttggattcggccttagccccctgagatgcactggttgatgatggtttagaagacaacacagcagaatgactcgaatgatggatggaatctgagtgactgggagaagctttcttctcttcatagtgtgtgtactcgctgactatgtccatgtcagagcaggcttccagttcatcagacaggaaagaggtgctgctgggagagcggtgggagtcagacaaggcatggctgctggagggtgtgagggaccgagcatccagcttggcctgcaggacttcaatcactttctccttctcctgcagctccctgctgagcctgagggccagtggctcaagtccagcttgatctttctcacttttatgatccttggtgctgagtttgctggtgagcctctctgtcagctggcttccctgggcgagttgctcccggaagctctgtcccaggtagtagtcaatgtcattgctccttaggagatcctcaaaagattttactgtatcttttgcatgccgggtgataagataacaaatacctctcccttctcgtattttttgccgtaggtaagacagttcccgggcctgatcctgaatcagggaatcatatttcccaggccacgaggctgatctcagctcctcagccagcttctcttctagtccattttttgggagctgggcctccagctgggatactctctggatgagactctccaggtcctttttggcctgaagccctggagagtagaaagccccagtgccatcagacagccacccctcatcctcatcagggacactatgaggtgaagacccctccaaggtgccaacagctctcagcttccggggtctttccagactagacgaataatcacttgtaactgagagggaccggacccggctcttgaggttttgaatgaccttgttggcattctgcagctgggccttcagatctttgatgtcctttcgtaggaccaagatgttttctgactttccatatacccggaactcttcctgcttccctagctggttctccaagggcttcctctcagaggaactagccagtgttgagccccggcgtccctgctcagagcacagcccctccatcaggaccatttccttgaggctgttgtgctcctcacactcaggactggtggtttcctcccgttcagcctcattctcgcttcggccacaagtctcatagcccaggtcctggaggtccacctggatctgcttgctgtcctgcttcaccaaggattcacctgtaagcataactctgtatttctccagctcgttagcctgagcaaagacagtggcttctgatagcagcagcttctcctggagatcttgatagcgttgtttgcattgtgacagctgggagcgcaggtgctgggtggaccctggtaggctaaacgctgactgaggcccagggtcacgaggctgggactggttatccaattggtgggcatccactgtgaaggtagccccaaggtcaaggctctggggtctggggaaaggcctcacagtcacattcccctcctcttggtgttggtgcttcccaggggaaccaaccagttctgtgtttattctttcaatggtgctggtcagatgcacaaggagctctggagtaagtttactattcccttccttgctactcagcacaagttgttctttgaggaggttgatgatattgtgggcattcttcagttttccctggagctttctgaactcagcctgaaggctactctcactcagaccctctttggttaccacagtctcaaccatcacctcgcccttctccttgtcttcctcgatctcccatccatcagacattgcttctcccatctgctctttcagctccgcattctcaaggcaaaggctcagcatggtgttcctgatgtgggacactgaggagaatcctgcttcctcaatttgagcctttagctccttcagttcctcctcagctttcctcttctcttctaagtgctggtggaactcagccctcaggtggagcatttcttcctgaagacacctgttactgtcccctcccatcggagaaggaggggaaaaagatgggttctgggtctccacagttgccagacttttctccaaagccaccttgacaagttgctggtgactatggtgtgcagcctcctcctcaatactgtcagtgaactcagtgcttgtatcttcggtgtcatcccctgcagctgcacctccaatggcggccagggtctccagcctgtttaagcgctccaagcttcttccaagaacttcttctagccgactgcgtaacacctgagccccttccagttccacctgcagagttcggtctctctcagagctctctggatgggcatggaacttcaccagactgctatagagctgtctctctgcttgtaaggcctcattgagccgactccgttcatctactagtccttctagcatcagcagcaactgttgtcttcggtttcctgaaatttcttgaccctgggattctactgaagcaactttttcccgaagaagtaagacttcctgggtcaggcgttccatagctggtatgtcttcaggatcaaccagttgcatttgcaggtcctttatgagatcttctttaatctgtatgttcctggtcagagactccatatcagcagcctgcacctgcagctcttcttcctgcacagccatcatggactgtagagcagaaagttccatctgactttctctttcttttttagccatgagttcaagttcctctttggcattactcagttctttttccagccctgcaactgtgtccaagtctcctaatgtggatctgggtatgctgacatcctctttggcagtcaatgaagtgctatcatctctggaaggtatctgcattgaaccttgatcagtctgttttccaagacggccagtgggggtaacttcagcttgttggttagagatgggtgcttgggacatcagggagtctctccctcctaaatattggcgcagggcctgtaattctgaatttctttccattaaggcttgcaccaacttctctgcagcagcttggctttcctgctccctggtgctcacagactgaagcaggccttgaatctccatttcatgttccagcacttgtttatttcgatcacttagaaggtcctgcagcatcctttcctttcgctgtagacgctggcacagctcctctgctatctcactctgccctggtccaagtttgcagagcagtgttgcactaagatcctccacttctttgttcctatcatgaagagacgtctgtaactgctgaatgatactctcttgttccttctgccaacggctaaatttggtttccatttcttctttcagccactggaggttttgacaggtagtagataactgttccacttccaggcctttggccctcaggagactctccatactttgcatagtagcttcattggaggagaggacatcgcgcagtctctctaagtcatgatctcgctctctcacagcaagacgaagctggcgcagttctttttctttctcttctagagcagagaatttttcatctatagcccgctccagagcaacagctttatcatgtattcgctggcgaagtttctcaagcaacatttcatttgcttcaagggttttgtctgagttatctcgatactgtaggagctcccgaaattcctgaagcaactgctccttgtgactcagactatggtttaggtgctggatgttttgttcctgggttcgaatctcattgtatttttcagcctcccaggcacgaagctgttggctcttattctgcaattcttcttgtagctgctgcaaggcttttcgcaattcctggttatgtttccaagaagcctctttctgctgttcactctcgtgtgctgcagcctctacaaattgcacacattgtttggcatcagccagttggcgctctttctgtcgtaccaccctctggagcttctgtatttcaagttggctgcagaataaagcactctgaagatcaagcagagctacctgttgctgagctggagaagtaccctctgagctgtgaagttgtccaagctggctttggtgcagcatttctcgaagctttgccattgtgtcattttgaccttcaattacctggtacaactcctcagtctcacgttccctgcttttcagagtttccttgaggttctgaattgtaccatcttgcttttgagacgactcctgagcacactttagttcatagctcatttcattaagtttctcttgaagaatcttgttggtggcctctgtttgctggattttttcctggagttctgccaagtgggaatcagatacagactgctgagttatagtggtctcatgtgaattcagcttttgttgtttcagcaactcttcagtcatgggctgcacttccatgctagttggctcctccaacagatgtagcagttgttgtttctcccgagatagctgttctacaagcctctcctgggcagccaggctctgattcagttcttcaattctcttgtccctctgggccagggcctcagtgtattggtcgggcttgacctggtctcctggtacatcttcccagtttttggtgactcccttcagtttctctgagagctccaggttacactccttctctgcttccaccagagctgccatccgcgcagcttcattctttgctagcctggattcctcctgcagaagctggatcttattctccaagagctcataaacatgctccgtctcctgctgtcgctcctcaaactggcgtcggagctcagcttcattctgactgttgagattctccacatcagcccatgttttatccagatgctgtttcttgtcctggagttctcgtttcaagctctccacttcaaccttcagctcaatgttccgcttgtagatgtcctcccggctggcctcatacttctgttgcatgcgctcctccaggaagtagatgcgcagcttgaggctgaagttctccttcttcaggtcattgaggtgcttctcaaagtctcgaagagcctgggtctgtacctgagggggtttctcaaatgctctcaaggaatatgtctgcacaaacgggaccttttcaccacttctccagatctgtgactgcactggagggcctcgatctttagtgtcactaagaaaagctgctgtgtgactcgttctgggtaccatctccccatcatcctctgcaaaataatctctcgtccaggtctgctccattttccaggctctttccttagtctcaggacgctcctcacccgggaggggaagcagcctgggaaaatgagaagccttgcccacgaatctccagcgcaaaaggcagcagctttttcctccccagctcctttctgcgtcggcggcgaagagagagctctgctccctgcttttttagaaaatggatttgacgtggccgaacctgcggctagccgtgcgacccgcacaagggagggactgttctcagtaggaggctggactcagagcggcgcggcgcccggggctgtttcgtgagctggagccagcggctgcccgggccgcggtgcgcgcactctccaggctgagacacgactg

SEQ ID NO: 8812 - RNA, 7753 nt, Homo sapiens
  source 1..7753: mol_type = other RNA
aagtgtgcagggcactggtgctgctccgaagctcatgaatacctttgctgcctagcacctctgtgccttgggcttcaaggccagggaagctgcacgctgatctcacaagagacactatctttttgaccagcagcttgccctccgcaatctgctgtcttagggcactgtagtcatcaatgtggccaatgacatggcggccatgcttattggcaaaggagccatcagtagcatcaccctctagcttgggaggggtcttcattactggagaagtatccaaacccaagccatttgctctgttgattatgggcgtttctgagccaggagtagaggaagcagagctggggaagaccagagctggggaattcataccaacatcccggactggaggggacacagctgaatcttggaggagcagctgcttgtttccagggtcagtgctggctgggaagttctggttaatggaggaggggctgaggctggctttgccagcaccgctctccagctgctgttgcagctgcagtcgcagacaattgttcccctgaatgctctgctccagctgccctctcagagctcgtacctctgccaccaggtggctcaggtcactgctcaaagggatttggtgacaggcatccaggctgtaagctttcagccccttcttggaattgccataaagtgcctcgtagatttgtagctctgactggagggactcaaagagctgctgtttctcttcacactgttgctgcaggagaaccagcttgtgctgcagtctggagtcgttttcctggagggaaagacgttcctccctgaaatgcaagacctcttgctgcttctccctcaagtcttccaaaagctgctgcctttccaccttctggtgctccagctccttttccagctcttgaaggtgggatcgagaggacagcagagcctccctcaggctttctgtttcctgggagtgctctctggaaacatgactcagttgagcctgaagtcttcgattgtcttccctgaggactctgttctcattgcagagctgaggtatggactccaggccctgactgtagaagttagaagtggatccccttccacgagcagtagaggtcagccggtgttccagttgctcccgtaggcggtcattgatgcagatggattcctccaggcgctggcgcaggttccggatttcaccaagatgctcttccagcaggtcagcccctgtgggtttggagttaagctggtacacagaggagcctgaggataggtccccagatacactccctttctgaggcctcatcacatcccacttgccactgctgcccaggtacccaggctctaggattcttcccagttctatggtgccccttggaggagagtgaggctgggcagagttgaggtagtaggaagagtcggcttccaagtcgttgctcagcaatgtagctgtggaagcaggaggaacagtgctggcactttctcccaactgcttctgcagcatctgtagctcctgctgagcctcagccaaggagaccactggtgtctcacagcagccaaggaggagagggccagtggggctgaaaggcaggaagctggatggagctgagggcaatggtgcctgaggaaggctagccagcttgggtatggagtgaaaatgaaagcctgaatgggcctggttggcctccttgggggtattctggggagttggcaagctgatggggttgctgttggattcggccttagccccctgagatgcactggttgatgatggtttagaagacaacacagcagaatgactcgaatgatggatggaatctgagtgactgggagaagctttcttctcttcatagtgtgtgtactcgctgactatgtccatgtcagagcaggcttccagttcatcagacaggaaagaggtgctgctgggagagcggtgggagtcagacaaggcatggctgctggagggtgtgagggaccgagcatccagcttggcctgcaggacttcaatcactttctccttctcctgcagctccctgctgagcctgagggccagtggctcaagtccagcttgatctttctcacttttatgatccttggtgctgagtttgctggtgagcctctctgtcagctggcttccctgggcgagttgctcccggaagctctgtcccaggtagtagtcaatgtcattgctccttaggagatcctcaaaagattttactgtatcttttgcatgccgggtgataagataacaaatacctctcccttctcgtattttttgccgtaggtaagacagttcccgggcctgatcctgaatcagggaatcatatttcccaggccacgaggctgatctcagctcctcagccagcttctcttctagtccattttttgggagctgggcctccagctgggatactctctggatgagactctccaggtcctttttggcctgaagccctggagagtagaaagccccagtgccatcagacagccacccctcatcctcatcagggacactatgaggtgaagacccctccaaggtgccaacagctctcagcttccggggtctttccagactagacgaataatcacttgtaactgagagggaccggacccggctcttgaggttttgaatgaccttgttggcattctgcagctgggccttcagatctttgatgtcctttcgtaggaccaagatgttttctgactttccatatacccggaactcttcctgcttccctagctggttctccaagggcttcctctcagaggaactagccagtgttgagccccggcgtccctgctcagagcacagcccctccatcaggaccatttccttgaggctgttgtgctcctcacactcaggactggtggtttcctcccgttcagcctcattctcgcttcggccacaagtctcatagcccaggtcctggaggtccacctggatctgcttgctgtcctgcttcaccaaggattcacctgtaagcataactctgtatttctccagctcgttagcctgagcaaagacagtggcttctgatagcagcagcttctcctggagatcttgatagcgttgtttgcattgtgacagctgggagcgcaggtgctgggtggaccctggtaggctaaacgctgactgaggcccagggtcacgaggctgggactggttatccaattggtgggcatccactgtgaaggtagccccaaggtcaaggctctggggtctggggaaaggcctcacagtcacattcccctcctcttggtgttggtgcttcccaggggaaccaaccagttctgtgtttattctttcaatggtgctggtcagatgcacaaggagctctggagtaagtttactattcccttccttgctactcagcacaagttgttctttgaggaggttgatgatattgtgggcattcttcagttttccctggagctttctgaactcagcctgaaggctactctcactcagaccctctttggttaccacagtctcaaccatcacctcgcccttctccttgtcttcctcgatctcccatccatcagacattgcttctcccatctgctctttcagctccgcattctcaaggcaaaggctcagcatggtgttcctgatgtgggacactgaggagaatcctgcttcctcaatttgagcctttagctccttcagttcctcctcagctttcctcttctcttctaagtgctggtggaactcagccctcaggtggagcatttcttcctgaagacacctgttactgtcccctcccatcggagaaggaggggaaaaagatgggttctgggtctccacagttgccagacttttctccaaagccaccttgacaagttgctggtgactatggtgtgcagcctcctcctcaatactgtcagtgaactcagtgcttgtatcttcggtgtcatcccctgcagctgcacctccaatggcggccagggtctccagcctgtttaagcgctccaagcttcttccaagaacttcttctagccgactgcgtaacacctgagccccttccagttccacctgcagagttcggtctctctcagagctctctggatgggcatggaacttcaccagactgctatagagctgtctctctgcttgtaaggcctcattgagccgactccgttcatctactagtccttctagcatcagcagcaactgttgtcttcggtttcctgaaatttcttgaccctgggattctactgaagcaactttttcccgaagaagtaagacttcctgggtcaggcgttccatagctggtatgtcttcaggatcaaccagttgcatttgcaggtcctttatgagatcttctttaatctgtatgttcctggtcagagactccatatcagcagcctgcacctgcagctcttcttcctgcacagccatcatggactgtagagcagaaagttccatctgactttctctttcttttttagccatgagttcaagttcctctttggcattactcagttctttttccagccctgcaactgtgtccaagtctcctaatgtggatctgggtatgctgacatcctctttggcagtcaatgaagtgctatcatctctggaaggtatctgcattgaaccttgatcagtctgttttccaagacggccagtgggggtaacttcagcttgttggttagagatgggtgcttgggacatcagggagtctctccctcctaaatattggcgcagggcctgtaattctgaatttctttccattaaggcttgcaccaacttctctgcagcagcttggctttcctgctccctggtgctcacagactgaagcaggccttgaatctccatttcatgttccagcacttgtttatttcgatcacttagaaggtcctgcagcatcctttcctttcgctgtagacgctggcacagctcctctgctatctcactctgccctggtccaagtttgcagagcagtgttgcactaagatcctccacttctttgttcctatcatgaagagacgtctgtaactgctgaatgatactctcttgttccttctgccaacggctaaatttggtttccatttcttctttcagccactggaggttttgacaggtagtagataactgttccacttccaggcctttggccctcaggagactctccatactttgcatagtagcttcattggaggagaggacatcgcgcagtctctctaagtcatgatctcgctctctcacagcaagacgaagctggcgcagttctttttctttctcttctagagcagagaatttttcatctatagcccgctccagagcaacagctttatcatgtattcgctggcgaagtttctcaagcaacatttcatttgcttcaagggttttgtctgagttatctcgatactgtaggagctcccgaaattcctgaagcaactgctccttgtgactcagactatggtttaggtgctggatgttttgttcctgggttcgaatctcattgtatttttcagcctcccaggcacgaagctgttggctcttattctgcaattcttcttgtagctgctgcaaggcttttcgcaattcctggttatgtttccaagaagcctctttctgctgttcactctcgtgtgctgcagcctctacaaattgcacacattgtttggcatcagccagttggcgctctttctgtcgtaccaccctctggagcttctgtatttcaagttggctgcagaataaagcactctgaagatcaagcagagctacctgttgctgagctggagaagtaccctctgagctgtgaagttgtccaagctggctttggtgcagcatttctcgaagctttgccattgtgtcattttgaccttcaattacctggtacaactcctcagtctcacgttccctgcttttcagagtttccttgaggttctgaattgtaccatcttgcttttgagacgactcctgagcacactttagttcatagctcatttcattaagtttctcttgaagaatcttgttggtggcctctgtttgctggattttttcctggagttctgccaagtgggaatcagatacagactgctgagttatagtggtctcatgtgaattcagcttttgttgtttcagcaactcttcagtcatgggctgcacttccatgctagttggctcctccaacagatgtagcagttgttgtttctcccgagatagctgttctacaagcctctcctgggcagccaggctctgattcagttcttcaattctcttgtccctctgggccagggcctcagtgtattggtcgggcttgacctggtctcctggtacatcttcccagtttttggtgactcccttcagtttctctgagagctccaggttacactccttctctgcttccaccagagctgccatccgcgcagcttcattctttgctagcctggattcctcctgcagaagctggatcttattctccaagagctcataaacatgctccgtctcctgctgtcgctcctcaaactggcgtcggagctcagcttcattctgactgttgagattctccacatcagcccatgttttatccagatgctgtttcttgtcctggagttctcgtttcaagctctccacttcaaccttcagctcaatgttccgcttgtagatgtcctcccggctggcctcatacttctgttgcatgcgctcctccaggaagtagatgcgcagcttgaggctgaagttctccttcttcaggtcattgaggtgcttctcaaagtctcgaagagcctgggtctgtacctgagggggtttctcaaatgctctcaaggaatatgtctgcacaaacgggaccttttcaccacttctccagatctgtgactgcactggagggcctcgatctttagtgtcactaagaaaagcttctttccttcgttctgccaacttgccagaaggagcccaagaaaaagcacccagatgcttcagtcaacttcttagaattcttcttttttttatgttcagaaaagatggaaattcatttctgctgtgtgactcgttctgggtaccatctccccatcatcctctgcaaaataatctctcgtccaggtctgctccattttccaggctctttccttagtctcaggacgctcctcacccgggaggggaagcagcctgggaaaatgagaagccttgcccacgaatctccagcgcaaaaggcagcagctttttcctccccagctcctttctgcgtcggcggcgaagagagagctctgctccctgcttttttagaaaatggatttgacgtggccgaacctgcggctagccgtgcgacccgcacaagggagggactgttctcagtaggaggctggactcagagcggcgcggcgcccggggctgtttcgtgagctggagccagcggctgcccgggccgcggtgcgcgcactctccaggctgagacacgactggctggcacgagttgctcggcaccagctgagctgtcaaccgcgagcggaggcggggctcccgacaaccagtgtgctggggcagaatcggcccaggttacacgccccctgaaccaccctcgcgtctccccgacccctctctcgctggctcagatgaatgatgacggcagagggcagagagcttagaggacgcggtaccaagccccgtccctcgcccatcccaacgaaggtcttagaatacaatcaaccaactacaggaagaatttgtagaggaggttttcttgtgtgtctgcatcgccccacccacaggtaaccccagagccagagatggagtctaggaaggtttaggagcaatcccggctga

SEQ ID NO: 8813 - RNA, 6637 nt, Homo sapiens
  source 1..6637: mol_type = other RNA
aagtgtgcagggcactggtgctgctccgaagctcatgaatacctttgctgcctagcacctctgtgccttgggcttcaaggccagggaagctgcacgctgatctcacaagagacactatctttttgaccagcagcttgccctccgcaatctgctgtcttagggcactgtagtcatcaatgtggccaatgacatggcggccatgcttattggcaaaggagccatcagtagcatcaccctctagcttgggaggggtcttcattactggagaagtatccaaacccaagccatttgctctgttgattatgggcgtttctgagccaggagtagaggaagcagagctggggaagaccagagctggggaattcataccaacatcccggactggaggggacacagctgaatcttggaggagcagctgcttgtttccagggtcagtgctggctgggaagttctggttaatggaggaggggctgaggctggctttgccagcaccgctctccagctgctgttgcagctgcagtcgcagacaattgttcccctgaatgctctgctccagctgccctctcagagctcgtacctctgccaccaggtggctcaggtcactgctcaaagggatttggtgacaggcatccaggctgtaagctttcagccccttcttggaattgccataaagtgcctcgtagatttgtagctctgactggagggactcaaagagctgctgtttctcttcacactgttgctgcaggagaaccagcttgtgctgcagtctggagtcgttttcctggagggaaagacgttcctccctgaaatgcaagacctcttgctgcttctccctcaagtcttccaaaagctgctgcctttccaccttctggtgctccagctccttttccagctcttgaaggtgggatcgagaggacagcagagcctccctcaggctttctgtttcctgggagtgctctctggaaacatgactcagttgagcctgaagtcttcgattgtcttccctgaggactctgttctcattgcagagctgaggtatggactccaggccctgactgtagaagttagaagtggatccccttccacgagcagtagaggtcagccggtgttccagttgctcccgtaggcggtcattgatgcagatggattcctccaggcgctggcgcaggttccggatttcaccaagatgctcttccagcaggtcagcccctgtgggtttggagttaagctggtacacagaggagcctgaggataggtccccagatacactccctttctgaggcctcatcacatcccacttgccactgctgcccaggtacccaggctctaggattcttcccagttctatggtgccccttggaggagagtgaggctgggcagagttgaggtagtaggaagagtcggcttccaagtcgttgctcagcaatgtagctgtggaagcaggaggaacagtgctggcactttctcccaactgcttctgcagcatctgtagctcctgctgagcctcagccaaggagaccactggtgtctcacagcagccaaggaggagagggccagtggggctgaaaggcaggaagctggatggagctgagggcaatggtgcctgaggaaggctagccagcttgggtatggagtgaaaatgaaagcctgaatgggcctggttggcctccttgggggtattctggggagttggcaagctgatggggttgctgttggattcggccttagccccctgagatgcactggttgatgatggtttagaagacaacacagcagaatgactcgaatgatggatggaatctgagtgactgggagaagctttcttctcttcatagtgtgtgtactcgctgactatgtccatgtcagagcaggcttccagttcatcagacaggaaagaggtgctgctgggagagcggtgggagtcagacaaggcatggctgctggagggtgtgagggaccgagcatccagcttggcctgcaggacttcaatcactttctccttctcctgcagctccctgctgagcctgagggccagtggctcaagtccagcttgatctttctcacttttatgatccttggtgctgagtttgctggtgagcctctctgtcagctggcttccctgggcgagttgctcccggaagctctgtcccaggtagtagtcaatgtcattgctccttaggagatcctcaaaagattttactgtatcttttgcatgccgggtgataagataacaaatacctctcccttctcgtattttttgccgtaggtaagacagttcccgggcctgatcctgaatcagggaatcatatttcccaggccacgaggctgatctcagctcctcagccagcttctcttctagtccattttttgggagctgggcctccagctgggatactctctggatgagactctccaggtcctttttggcctgaagccctggagagtagaaagccccagtgccatcagacagccacccctcatcctcatcagggacactatgaggtgaagacccctccaaggtgccaacagctctcagcttccggggtctttccagactagacgaataatcacttgtaactgagagggaccggacccggctcttgaggttttgaatgaccttgttggcattctgcagctgggccttcagatctttgatgtcctttcgtaggaccaagatgttttctgactttccatatacccggaactcttcctgcttccctagctggttctccaagggcttcctctcagaggaactagccagtgttgagccccggcgtccctgctcagagcacagcccctccatcaggaccatttccttgaggctgttgtgctcctcacactcaggactggtggtttcctcccgttcagcctcattctcgcttcggccacaagtctcatagcccaggtcctggaggtccacctggatctgcttgctgtcctgcttcaccaaggattcacctgtaagcataactctgtatttctccagctcgttagcctgagcaaagacagtggcttctgatagcagcagcttctcctggagatcttgatagcgttgtttgcattgtgacagctgggagcgcaggtgctgggtggaccctggtaggctaaacgctgactgaggcccagggtcacgaggctgggactggttatccaattggtgggcatccactgtgaaggtagccccaaggtcaaggctctggggtctggggaaaggcctcacagtcacattcccctcctcttggtgttggtgcttcccaggggaaccaaccagttctgtgtttattctttcaatggtgctggtcagatgcacaaggagctctggagtaagtttactattcccttccttgctactcagcacaagttgttctttgaggaggttgatgatattgtgggcattcttcagttttccctggagctttctgaactcagcctgaaggctactctcactcagaccctctttggttaccacagtctcaaccatcacctcgcccttctccttgtcttcctcgatctcccatccatcagacattgcttctcccatctgctctttcagctccgcattctcaaggcaaaggctcagcatggtgttcctgatgtgggacactgaggagaatcctgcttcctcaatttgagcctttagctccttcagttcctcctcagctttcctcttctcttctaagtgctggtggaactcagccctcaggtggagcatttcttcctgaagacacctgttactgtcccctcccatcggagaaggaggggaaaaagatgggttctgggtctccacagttgccagacttttctccaaagccaccttgacaagttgctggtgactatggtgtgcagcctcctcctcaatactgtcagtgaactcagtgcttgtatcttcggtgtcatcccctgcagctgcacctccaatggcggccagggtctccagcctgtttaagcgctccaagcttcttccaagaacttcttctagccgactgcgtaacacctgagccccttccagttccacctgcagagttcggtctctctcagagctctctggatgggcatggaacttcaccagactgctatagagctgtctctctgcttgtaaggcctcattgagccgactccgttcatctactagtccttctagcatcagcagcaactgttgtcttcggtttcctgaaatttcttgaccctgggattctactgaagcaactttttcccgaagaagtaagacttcctgggtcaggcgttccatagctggtatgtcttcaggatcaaccagttgcatttgcaggtcctttatgagatcttctttaatctgtatgttcctggtcagagactccatatcagcagcctgcacctgcagctcttcttcctgcacagccatcatggactgtagagcagaaagttccatctgactttctctttcttttttagccatgagttcaagttcctctttggcattactcagttctttttccagccctgcaactgtgtccaagtctcctaatgtggatctgggtatgctgacatcctctttggcagtcaatgaagtgctatcatctctggaaggtatctgcattgaaccttgatcagtctgttttccaagacggccagtgggggtaacttcagcttgttggttagagatgggtgcttgggacatcagggagtctctccctcctaaatattggcgcagggcctgtaattctgaatttctttccattaaggcttgcaccaacttctctgcagcagcttggctttcctgctccctggtgctcacagactgaagcaggccttgaatctccatttcatgttccagcacttgtttatttcgatcacttagaaggtcctgcagcatcctttcctttcgctgtagacgctggcacagctcctctgctatctcactctgccctggtccaagtttgcagagcagtgttgcactaagatcctccacttctttgttcctatcatgaagagacgtctgtaactgctgaatgatactctcttgttccttctgccaacggctaaatttggtttccatttcttctttcagccactggaggttttgacaggtagtagataactgttccacttccaggcctttggccctcaggagactctccatactttgcatagtagcttcattggaggagaggacatcgcgcagtctctctaagtcatgatctcgctctctcacagcaagacgaagctggcgcagttctttttctttctcttctagagcagagaatttttcatctatagcccgctccagagcaacagctttatcatgtattcgctggcgaagtttctcaagcaacatttcatttgcttcaagggttttgtctgagttatctcgatactgtaggagctcccgaaattcctgaagcaactgctccttgtgactcagactatggtttaggtgctggatgttttgttcctgggttcgaatctcattgtatttttcagcctcccaggcacgaagctgttggctcttattctgcaattcttcttgtagctgctgcaaggcttttcgcaattcctggttatgtttccaagaagcctctttctgctgttcactctcgtgtgctgcagcctctacaaattgcacacattgtttggcatcagccagttggcgctctttctgtcgtaccaccctctggagcttctgtatttcaagttggctgcagaataaagcactctgaagatcaagcagagctacctgttgctgagctggagaagtaccctctgagctgtgaagttgtccaagctggctttggtgcagcatttctcgaagctttgccattgtgtcattttgaccttcaattacctggtacaactcctcagtctcacgttccctgcttttcagagtttccttgaggttctgaattgtaccatcttgcttttgagacgactcctgagcacactttagttcatagctcatttcattaagtttctcttgaagaatcttgttggtggcctctgtttgctggattttttcctggagttctgccaagtgggaatcagatacagactgctgagttatagtggtctcatgtgaattcagcttttgttgtttcagcaactcttcagtcatgggctgcacttccatgctagttggctcctccaacagatgtagcagttgttgtttctcccgagatagctgttctacaagcctctcctgggcagccaggctctgattcagttcttcaattctcttgtccctctgggccagggcctcagtgtattggtcgggcttgacctggtctcctggtacatcttcccagtttttggtgactcccttcagtttctctgagagctccaggttacactccttctctgcttccaccagagctgccatccgcgcagcttcattctttgctagcctggattcctcctgcagaagctggatcttattctccaagagctcataaacatgctccgtctcctgctgtcgctcctcaaactggcgtcggagctcagcttcattctgactgttgagattctccacatcagccccgcttgtagatgtcctcccggctggcctcatacttctgttgcatgcgctcctccaggaagtagatgcgcagcttgaggctgaagttctccttcttcaggtcattgaggtgctcagggagatatttgc

SEQ ID NO: 8814 - RNA, 7297 nt, Homo sapiens
  source 1..7297: mol_type = other RNA
aagtgtgcagggcactggtgctgctccgaagctcatgaatacctttgctgcctagcacctctgtgccttgggcttcaaggccagggaagctgcacgctgatctcacaagagacactatctttttgaccagcagcttgccctccgcaatctgctgtcttagggcactgtagtcatcaatgtggccaatgacatggcggccatgcttattggcaaaggagccatcagtagcatcaccctctagcttgggaggggtcttcattactggagaagtatccaaacccaagccatttgctctgttgattatgggcgtttctgagccaggagtagaggaagcagagctggggaagaccagagctggggaattcataccaacatcccggactggaggggacacagctgaatcttggaggagcagctgcttgtttccagggtcagtgctggctgggaagttctggttaatggaggaggggctgaggctggctttgccagcaccgctctccagctgctgttgcagctgcagtcgcagacaattgttcccctgaatgctctgctccagctgccctctcagagctcgtacctctgccaccaggtggctcaggtcactgctcaaagggatttggtgacaggcatccaggctgtaagctttcagccccttcttggaattgccataaagtgcctcgtagatttgtagctctgactggagggactcaaagagctgctgtttctcttcacactgttgctgcaggagaaccagcttgtgctgcagtctggagtcgttttcctggagggaaagacgttcctccctgaaatgcaagacctcttgctgcttctccctcaagtcttccaaaagctgctgcctttccaccttctggtgctccagctccttttccagctcttgaaggtgggatcgagaggacagcagagcctccctcaggctttctgtttcctgggagtgctctctggaaacatgactcagttgagcctgaagtcttcgattgtcttccctgaggactctgttctcattgcagagctgaggtatggactccaggccctgactgtagaagttagaagtggatccccttccacgagcagtagaggtcagccggtgttccagttgctcccgtaggcggtcattgatgcagatggattcctccaggcgctggcgcaggttccggatttcaccaagatgctcttccagcaggtcagcccctgtgggtttggagttaagctggtacacagaggagcctgaggataggtccccagatacactccctttctgaggcctcatcacatcccacttgccactgctgcccaggtacccaggctctaggattcttcccagttctatggtgccccttggaggagagtgaggctgggcagagttgaggtagtaggaagagtcggcttccaagtcgttgctcagcaatgtagctgtggaagcaggaggaacagtgctggcactttctcccaactgcttctgcagcatctgtagctcctgctgagcctcagccaaggagaccactggtgtctcacagcagccaaggaggagagggccagtggggctgaaaggcaggaagctggatggagctgagggcaatggtgcctgaggaaggctagccagcttgggtatggagtgaaaatgaaagcctgaatgggcctggttggcctccttgggggtattctggggagttggcaagctgatggggttgctgttggattcggccttagccccctgagatgcactggttgatgatggtttagaagacaacacagcagaatgactcgaatgatggatggaatctgagtgactgggagaagctttcttctcttcatagtgtgtgtactcgctgactatgtccatgtcagagcaggcttccagttcatcagacaggaaagaggtgctgctgggagagcggtgggagtcagacaaggcatggctgctggagggtgtgagggaccgagcatccagcttggcctgcaggacttcaatcactttctccttctcctgcagctccctgctgagcctgagggccagtggctcaagtccagcttgatctttctcacttttatgatccttggtgctgagtttgctggtgagcctctctgtcagctggcttccctgggcgagttgctcccggaagctctgtcccaggtagtagtcaatgtcattgctccttaggagatcctcaaaagattttactgtatcttttgcatgccgggtgataagataacaaatacctctcccttctcgtattttttgccgtaggtaagacagttcccgggcctgatcctgaatcagggaatcatatttcccaggccacgaggctgatctcagctcctcagccagcttctcttctagtccattttttgggagctgggcctccagctgggatactctctggatgagactctccaggtcctttttggcctgaagccctggagagtagaaagccccagtgccatcagacagccacccctcatcctcatcagggacactatgaggtgaagacccctccaaggtgccaacagctctcagcttccggggtctttccagactagacgaataatcacttgtaactgagagggaccggacccggctcttgaggttttgaatgaccttgttggcattctgcagctgggccttcagatctttgatgtcctttcgtaggaccaagatgttttctgactttccatatacccggaactcttcctgcttccctagctggttctccaagggcttcctctcagaggaactagccagtgttgagccccggcgtccctgctcagagcacagcccctccatcaggaccatttccttgaggctgttgtgctcctcacactcaggactggtggtttcctcccgttcagcctcattctcgcttcggccacaagtctcatagcccaggtcctggaggtccacctggatctgcttgctgtcctgcttcaccaaggattcacctgtaagcataactctgtatttctccagctcgttagcctgagcaaagacagtggcttctgatagcagcagcttctcctggagatcttgatagcgttgtttgcattgtgacagctgggagcgcaggtgctgggtggaccctggtaggctaaacgctgactgaggcccagggtcacgaggctgggactggttatccaattggtgggcatccactgtgaaggtagccccaaggtcaaggctctggggtctggggaaaggcctcacagtcacattcccctcctcttggtgttggtgcttcccaggggaaccaaccagttctgtgtttattctttcaatggtgctggtcagatgcacaaggagctctggagtaagtttactattcccttccttgctactcagcacaagttgttctttgaggaggttgatgatattgtgggcattcttcagttttccctggagctttctgaactcagcctgaaggctactctcactcagaccctctttggttaccacagtctcaaccatcacctcgcccttctccttgtcttcctcgatctcccatccatcagacattgcttctcccatctgctctttcagctccgcattctcaaggcaaaggctcagcatggtgttcctgatgtgggacactgaggagaatcctgcttcctcaatttgagcctttagctccttcagttcctcctcagctttcctcttctcttctaagtgctggtggaactcagccctcaggtggagcatttcttcctgaagacacctgttactgtcccctcccatcggagaaggaggggaaaaagatgggttctgggtctccacagttgccagacttttctccaaagccaccttgacaagttgctggtgactatggtgtgcagcctcctcctcaatactgtcagtgaactcagtgcttgtatcttcggtgtcatcccctgcagctgcacctccaatggcggccagggtctccagcctgtttaagcgctccaagcttcttccaagaacttcttctagccgactgcgtaacacctgagccccttccagttccacctgcagagttcggtctctctcagagctctctggatgggcatggaacttcaccagactgctatagagctgtctctctgcttgtaaggcctcattgagccgactccgttcatctactagtccttctagcatcagcagcaactgttgtcttcggtttcctgaaatttcttgaccctgggattctactgaagcaactttttcccgaagaagtaagacttcctgggtcaggcgttccatagctggtatgtcttcaggatcaaccagttgcatttgcaggtcctttatgagatcttctttaatctgtatgttcctggtcagagactccatatcagcagcctgcacctgcagctcttcttcctgcacagccatcatggactgtagagcagaaagttccatctgactttctctttcttttttagccatgagttcaagttcctctttggcattactcagttctttttccagccctgcaactgtgtccaagtctcctaatgtggatctgggtatgctgacatcctctttggcagtcaatgaagtgctatcatctctggaaggtatctgcattgaaccttgatcagtctgttttccaagacggccagtgggggtaacttcagcttgttggttagagatgggtgcttgggacatcagggagtctctccctcctaaatattggcgcagggcctgtaattctgaatttctttccattaaggcttgcaccaacttctctgcagcagcttggctttcctgctccctggtgctcacagactgaagcaggccttgaatctccatttcatgttccagcacttgtttatttcgatcacttagaaggtcctgcagcatcctttcctttcgctgtagacgctggcacagctcctctgctatctcactctgccctggtccaagtttgcagagcagtgttgcactaagatcctccacttctttgttcctatcatgaagagacgtctgtaactgctgaatgatactctcttgttccttctgccaacggctaaatttggtttccatttcttctttcagccactggaggttttgacaggtagtagataactgttccacttccaggcctttggccctcaggagactctccatactttgcatagtagcttcattggaggagaggacatcgcgcagtctctctaagtcatgatctcgctctctcacagcaagacgaagctggcgcagttctttttctttctcttctagagcagagaatttttcatctatagcccgctccagagcaacagctttatcatgtattcgctggcgaagtttctcaagcaacatttcatttgcttcaagggttttgtctgagttatctcgatactgtaggagctcccgaaattcctgaagcaactgctccttgtgactcagactatggtttaggtgctggatgttttgttcctgggttcgaatctcattgtatttttcagcctcccaggcacgaagctgttggctcttattctgcaattcttcttgtagctgctgcaaggcttttcgcaattcctggttatgtttccaagaagcctctttctgctgttcactctcgtgtgctgcagcctctacaaattgcacacattgtttggcatcagccagttggcgctctttctgtcgtaccaccctctggagcttctgtatttcaagttggctgcagaataaagcactctgaagatcaagcagagctacctgttgctgagctggagaagtaccctctgagctgtgaagttgtccaagctggctttggtgcagcatttctcgaagctttgccattgtgtcattttgaccttcaattacctggtacaactcctcagtctcacgttccctgcttttcagagtttccttgaggttctgaattgtaccatcttgcttttgagacgactcctgagcacactttagttcatagctcatttcattaagtttctcttgaagaatcttgttggtggcctctgtttgctggattttttcctggagttctgccaagtgggaatcagatacagactgctgagttatagtggtctcatgtgaattcagcttttgttgtttcagcaactcttcagtcatgggctgcacttccatgctagttggctcctccaacagatgtagcagttgttgtttctcccgagatagctgttctacaagcctctcctgggcagccaggctctgattcagttcttcaattctcttgtccctctgggccagggcctcagtgtattggtcgggcttgacctggtctcctggtacatcttcccagtttttggtgactcccttcagtttctctgagagctccaggttacactccttctctgcttccaccagagctgccatccgcgcagcttcattctttgctagcctggattcctcctgcagaagctggatcttattctccaagagctcataaacatgctccgtctcctgctgtcgctcctcaaactggcgtcggagctcagcttcattctgactgttgagattctccacatcagccccgcttgtagatgtcctcccggctggcctcatacttctgttgcatgcgctcctccaggaagtagatgcgcagcttgaggctgaagttctccttcttcaggtcattgaggtgcttctcaaagtctcgaagagcctgggtctgtacctgagggggtttctcaaatgctctcaaggaatatgtctgcacaaacgggaccttttcaccacttctccagatctgtgactgcactggagggcctcgatctttagtgtcactaagaaaagcagaaggagcccaagaaaaagcacccagatgcttcagtcaacttcttagaattcttcttttttttatgttcagaaaagatggaaattcatttctgctgtgtgactcgttctgggtaccatctccccatcatcctctgcaaaataatctctcatccagggtgtggccgccgcagctgcttcttcctcctcggccgctgctgcccagctcccggctggctccgggcgccgtctttcccggctcggggtctgccgtggggactgaggggttcgcgtcgcgtccccggaccggtaaggcgtgtagtgagcccggcgggacgcgcgacagcagcagccaaagtcgcatcggcggcggcagcaggacccgctgtctgtgcccttcatggatttcctgggcctggccaccccagtcctagctacggttcctgcttgttttcctggtgttttccgggactgccagggcgcatcctctgggcctggctgagcatccccgtcagttccctgggcctcctccgcggctgcctctgc

SEQ ID NO: 8815 - RNA, 7180 nt, Homo sapiens
  source 1..7180: mol_type = other RNA
aagtgtgcagggcactggtgctgctccgaagctcatgaatacctttgctgcctagcacctctgtgccttgggcttcaaggccagggaagctgcacgctgatctcacaagagacactatctttttgaccagcagcttgccctccgcaatctgctgtcttagggcactgtagtcatcaatgtggccaatgacatggcggccatgcttattggcaaaggagccatcagtagcatcaccctctagcttgggaggggtcttcattactggagaagtatccaaacccaagccatttgctctgttgattatgggcgtttctgagccaggagtagaggaagcagagctggggaagaccagagctggggaattcataccaacatcccggactggaggggacacagctgaatcttggaggagcagctgcttgtttccagggtcagtgctggctgggaagttctggttaatggaggaggggctgaggctggctttgccagcaccgctctccagctgctgttgcagctgcagtcgcagacaattgttcccctgaatgctctgctccagctgccctctcagagctcgtacctctgccaccaggtggctcaggtcactgctcaaagggatttggtgacaggcatccaggctgtaagctttcagccccttcttggaattgccataaagtgcctcgtagatttgtagctctgactggagggactcaaagagctgctgtttctcttcacactgttgctgcaggagaaccagcttgtgctgcagtctggagtcgttttcctggagggaaagacgttcctccctgaaatgcaagacctcttgctgcttctccctcaagtcttccaaaagctgctgcctttccaccttctggtgctccagctccttttccagctcttgaaggtgggatcgagaggacagcagagcctccctcaggctttctgtttcctgggagtgctctctggaaacatgactcagttgagcctgaagtcttcgattgtcttccctgaggactctgttctcattgcagagctgaggtatggactccaggccctgactgtagaagttagaagtggatccccttccacgagcagtagaggtcagccggtgttccagttgctcccgtaggcggtcattgatgcagatggattcctccaggcgctggcgcaggttccggatttcaccaagatgctcttccagcaggtcagcccctgtgggtttggagttaagctggtacacagaggagcctgaggataggtccccagatacactccctttctgaggcctcatcacatcccacttgccactgctgcccaggtacccaggctctaggattcttcccagttctatggtgccccttggaggagagtgaggctgggcagagttgaggtagtaggaagagtcggcttccaagtcgttgctcagcaatgtagctgtggaagcaggaggaacagtgctggcactttctcccaactgcttctgcagcatctgtagctcctgctgagcctcagccaaggagaccactggtgtctcacagcagccaaggaggagagggccagtggggctgaaaggcaggaagctggatggagctgagggcaatggtgcctgaggaaggctagccagcttgggtatggagtgaaaatgaaagcctgaatgggcctggttggcctccttgggggtattctggggagttggcaagctgatggggttgctgttggattcggccttagccccctgagatgcactggttgatgatggtttagaagacaacacagcagaatgactcgaatgatggatggaatctgagtgactgggagaagctttcttctcttcatagtgtgtgtactcgctgactatgtccatgtcagagcaggcttccagttcatcagacaggaaagaggtgctgctgggagagcggtgggagtcagacaaggcatggctgctggagggtgtgagggaccgagcatccagcttggcctgcaggacttcaatcactttctccttctcctgcagctccctgctgagcctgagggccagtggctcaagtccagcttgatctttctcacttttatgatccttggtgctgagtttgctggtgagcctctctgtcagctggcttccctgggcgagttgctcccggaagctctgtcccaggtagtagtcaatgtcattgctccttaggagatcctcaaaagattttactgtatcttttgcatgccgggtgataagataacaaatacctctcccttctcgtattttttgccgtaggtaagacagttcccgggcctgatcctgaatcagggaatcatatttcccaggccacgaggctgatctcagctcctcagccagcttctcttctagtccattttttgggagctgggcctccagctgggatactctctggatgagactctccaggtcctttttggcctgaagccctggagagtagaaagccccagtgccatcagacagccacccctcatcctcatcagggacactatgaggtgaagacccctccaaggtgccaacagctctcagcttccggggtctttccagactagacgaataatcacttgtaactgagagggaccggacccggctcttgaggttttgaatgaccttgttggcattctgcagctgggccttcagatctttgatgtcctttcgtaggaccaagatgttttctgactttccatatacccggaactcttcctgcttccctagctggttctccaagggcttcctctcagaggaactagccagtgttgagccccggcgtccctgctcagagcacagcccctccatcaggaccatttccttgaggctgttgtgctcctcacactcaggactggtggtttcctcccgttcagcctcattctcgcttcggccacaagtctcatagcccaggtcctggaggtccacctggatctgcttgctgtcctgcttcaccaaggattcacctgtaagcataactctgtatttctccagctcgttagcctgagcaaagacagtggcttctgatagcagcagcttctcctggagatcttgatagcgttgtttgcattgtgacagctgggagcgcaggtgctgggtggaccctggtaggctaaacgctgactgaggcccagggtcacgaggctgggactggttatccaattggtgggcatccactgtgaaggtagccccaaggtcaaggctctggggtctggggaaaggcctcacagtcacattcccctcctcttggtgttggtgcttcccaggggaaccaaccagttctgtgtttattctttcaatggtgctggtcagatgcacaaggagctctggagtaagtttactattcccttccttgctactcagcacaagttgttctttgaggaggttgatgatattgtgggcattcttcagttttccctggagctttctgaactcagcctgaaggctactctcactcagaccctctttggttaccacagtctcaaccatcacctcgcccttctccttgtcttcctcgatctcccatccatcagacattgcttctcccatctgctctttcagctccgcattctcaaggcaaaggctcagcatggtgttcctgatgtgggacactgaggagaatcctgcttcctcaatttgagcctttagctccttcagttcctcctcagctttcctcttctcttctaagtgctggtggaactcagccctcaggtggagcatttcttcctgaagacacctgttactgtcccctcccatcggagaaggaggggaaaaagatgggttctgggtctccacagttgccagacttttctccaaagccaccttgacaagttgctggtgactatggtgtgcagcctcctcctcaatactgtcagtgaactcagtgcttgtatcttcggtgtcatcccctgcagctgcacctccaatggcggccagggtctccagcctgtttaagcgctccaagcttcttccaagaacttcttctagccgactgcgtaacacctgagccccttccagttccacctgcagagttcggtctctctcagagctctctggatgggcatggaacttcaccagactgctatagagctgtctctctgcttgtaaggcctcattgagccgactccgttcatctactagtccttctagcatcagcagcaactgttgtcttcggtttcctgaaatttcttgaccctgggattctactgaagcaactttttcccgaagaagtaagacttcctgggtcaggcgttccatagctggtatgtcttcaggatcaaccagttgcatttgcaggtcctttatgagatcttctttaatctgtatgttcctggtcagagactccatatcagcagcctgcacctgcagctcttcttcctgcacagccatcatggactgtagagcagaaagttccatctgactttctctttcttttttagccatgagttcaagttcctctttggcattactcagttctttttccagccctgcaactgtgtccaagtctcctaatgtggatctgggtatgctgacatcctctttggcagtcaatgaagtgctatcatctctggaaggtatctgcattgaaccttgatcagtctgttttccaagacggccagtgggggtaacttcagcttgttggttagagatgggtgcttgggacatcagggagtctctccctcctaaatattggcgcagggcctgtaattctgaatttctttccattaaggcttgcaccaacttctctgcagcagcttggctttcctgctccctggtgctcacagactgaagcaggccttgaatctccatttcatgttccagcacttgtttatttcgatcacttagaaggtcctgcagcatcctttcctttcgctgtagacgctggcacagctcctctgctatctcactctgccctggtccaagtttgcagagcagtgttgcactaagatcctccacttctttgttcctatcatgaagagacgtctgtaactgctgaatgatactctcttgttccttctgccaacggctaaatttggtttccatttcttctttcagccactggaggttttgacaggtagtagataactgttccacttccaggcctttggccctcaggagactctccatactttgcatagtagcttcattggaggagaggacatcgcgcagtctctctaagtcatgatctcgctctctcacagcaagacgaagctggcgcagttctttttctttctcttctagagcagagaatttttcatctatagcccgctccagagcaacagctttatcatgtattcgctggcgaagtttctcaagcaacatttcatttgcttcaagggttttgtctgagttatctcgatactgtaggagctcccgaaattcctgaagcaactgctccttgtgactcagactatggtttaggtgctggatgttttgttcctgggttcgaatctcattgtatttttcagcctcccaggcacgaagctgttggctcttattctgcaattcttcttgtagctgctgcaaggcttttcgcaattcctggttatgtttccaagaagcctctttctgctgttcactctcgtgtgctgcagcctctacaaattgcacacattgtttggcatcagccagttggcgctctttctgtcgtaccaccctctggagcttctgtatttcaagttggctgcagaataaagcactctgaagatcaagcagagctacctgttgctgagctggagaagtaccctctgagctgtgaagttgtccaagctggctttggtgcagcatttctcgaagctttgccattgtgtcattttgaccttcaattacctggtacaactcctcagtctcacgttccctgcttttcagagtttccttgaggttctgaattgtaccatcttgcttttgagacgactcctgagcacactttagttcatagctcatttcattaagtttctcttgaagaatcttgttggtggcctctgtttgctggattttttcctggagttctgccaagtgggaatcagatacagactgctgagttatagtggtctcatgtgaattcagcttttgttgtttcagcaactcttcagtcatgggctgcacttccatgctagttggctcctccaacagatgtagcagttgttgtttctcccgagatagctgttctacaagcctctcctgggcagccaggctctgattcagttcttcaattctcttgtccctctgggccagggcctcagtgtattggtcgggcttgacctggtctcctggtacatcttcccagtttttggtgactcccttcagtttctctgagagctccaggttacactccttctctgcttccaccagagctgccatccgcgcagcttcattctttgctagcctggattcctcctgcagaagctggatcttattctccaagagctcataaacatgctccgtctcctgctgtcgctcctcaaactggcgtcggagctcagcttcattctgactgttgagattctccacatcagccccgcttgtagatgtcctcccggctggcctcatacttctgttgcatgcgctcctccaggaagtagatgcgcagcttgaggctgaagttctccttcttcaggtcattgaggtgcttctcaaagtctcgaagagcctgggtctgtacctgagggggtttctcaaatgctctcaaggaatatgtctgcacaaacgggaccttttcaccacttctccagatctgtgactgcactggagggcctcgatctttagtgtcactaagaaaagctgctgtgtgactcgttctgggtaccatctccccatcatcctctgcaaaataatctctcatccagggtgtggccgccgcagctgcttcttcctcctcggccgctgctgcccagctcccggctggctccgggcgccgtctttcccggctcggggtctgccgtggggactgaggggttcgcgtcgcgtccccggaccggtaaggcgtgtagtgagcccggcgggacgcgcgacagcagcagccaaagtcgcatcggcggcggcagcaggacccgctgtctgtgcccttcatggatttcctgggcctggccaccccagtcctagctacggttcctgcttgttttcctggtgttttccgggactgccagggcgcatcctctgggcctggctgagcatccccgtcagttccct

SEQ ID NO: 8816 - RNA, 7199 nt, Homo sapiens
  source 1..7199: mol_type = other RNA
aagtgtgcagggcactggtgctgctccgaagctcatgaatacctttgctgcctagcacctctgtgccttgggcttcaaggccagggaagctgcacgctgatctcacaagagacactatctttttgaccagcagcttgccctccgcaatctgctgtcttagggcactgtagtcatcaatgtggccaatgacatggcggccatgcttattggcaaaggagccatcagtagcatcaccctctagcttgggaggggtcttcattactggagaagtatccaaacccaagccatttgctctgttgattatgggcgtttctgagccaggagtagaggaagcagagctggggaagaccagagctggggaattcataccaacatcccggactggaggggacacagctgaatcttggaggagcagctgcttgtttccagggtcagtgctggctgggaagttctggttaatggaggaggggctgaggctggctttgccagcaccgctctccagctgctgttgcagctgcagtcgcagacaattgttcccctgaatgctctgctccagctgccctctcagagctcgtacctctgccaccaggtggctcaggtcactgctcaaagggatttggtgacaggcatccaggctgtaagctttcagccccttcttggaattgccataaagtgcctcgtagatttgtagctctgactggagggactcaaagagctgctgtttctcttcacactgttgctgcaggagaaccagcttgtgctgcagtctggagtcgttttcctggagggaaagacgttcctccctgaaatgcaagacctcttgctgcttctccctcaagtcttccaaaagctgctgcctttccaccttctggtgctccagctccttttccagctcttgaaggtgggatcgagaggacagcagagcctccctcaggctttctgtttcctgggagtgctctctggaaacatgactcagttgagcctgaagtcttcgattgtcttccctgaggactctgttctcattgcagagctgaggtatggactccaggccctgactgtagaagttagaagtggatccccttccacgagcagtagaggtcagccggtgttccagttgctcccgtaggcggtcattgatgcagatggattcctccaggcgctggcgcaggttccggatttcaccaagatgctcttccagcaggtcagcccctgtgggtttggagttaagctggtacacagaggagcctgaggataggtccccagatacactccctttctgaggcctcatcacatcccacttgccactgctgcccaggtacccaggctctaggattcttcccagttctatggtgccccttggaggagagtgaggctgggcagagttgaggtagtaggaagagtcggcttccaagtcgttgctcagcaatgtagctgtggaagcaggaggaacagtgctggcactttctcccaactgcttctgcagcatctgtagctcctgctgagcctcagccaaggagaccactggtgtctcacagcagccaaggaggagagggccagtggggctgaaaggcaggaagctggatggagctgagggcaatggtgcctgaggaaggctagccagcttgggtatggagtgaaaatgaaagcctgaatgggcctggttggcctccttgggggtattctggggagttggcaagctgatggggttgctgttggattcggccttagccccctgagatgcactggttgatgatggtttagaagacaacacagcagaatgactcgaatgatggatggaatctgagtgactgggagaagctttcttctcttcatagtgtgtgtactcgctgactatgtccatgtcagagcaggcttccagttcatcagacaggaaagaggtgctgctgggagagcggtgggagtcagacaaggcatggctgctggagggtgtgagggaccgagcatccagcttggcctgcaggacttcaatcactttctccttctcctgcagctccctgctgagcctgagggccagtggctcaagtccagcttgatctttctcacttttatgatccttggtgctgagtttgctggtgagcctctctgtcagctggcttccctgggcgagttgctcccggaagctctgtcccaggtagtagtcaatgtcattgctccttaggagatcctcaaaagattttactgtatcttttgcatgccgggtgataagataacaaatacctctcccttctcgtattttttgccgtaggtaagacagttcccgggcctgatcctgaatcagggaatcatatttcccaggccacgaggctgatctcagctcctcagccagcttctcttctagtccattttttgggagctgggcctccagctgggatactctctggatgagactctccaggtcctttttggcctgaagccctggagagtagaaagccccagtgccatcagacagccacccctcatcctcatcagggacactatgaggtgaagacccctccaaggtgccaacagctctcagcttccggggtctttccagactagacgaataatcacttgtaactgagagggaccggacccggctcttgaggttttgaatgaccttgttggcattctgcagctgggccttcagatctttgatgtcctttcgtaggaccaagatgttttctgactttccatatacccggaactcttcctgcttccctagctggttctccaagggcttcctctcagaggaactagccagtgttgagccccggcgtccctgctcagagcacagcccctccatcaggaccatttccttgaggctgttgtgctcctcacactcaggactggtggtttcctcccgttcagcctcattctcgcttcggccacaagtctcatagcccaggtcctggaggtccacctggatctgcttgctgtcctgcttcaccaaggattcacctgtaagcataactctgtatttctccagctcgttagcctgagcaaagacagtggcttctgatagcagcagcttctcctggagatcttgatagcgttgtttgcattgtgacagctgggagcgcaggtgctgggtggaccctggtaggctaaacgctgactgaggcccagggtcacgaggctgggactggttatccaattggtgggcatccactgtgaaggtagccccaaggtcaaggctctggggtctggggaaaggcctcacagtcacattcccctcctcttggtgttggtgcttcccaggggaaccaaccagttctgtgtttattctttcaatggtgctggtcagatgcacaaggagctctggagtaagtttactattcccttccttgctactcagcacaagttgttctttgaggaggttgatgatattgtgggcattcttcagttttccctggagctttctgaactcagcctgaaggctactctcactcagaccctctttggttaccacagtctcaaccatcacctcgcccttctccttgtcttcctcgatctcccatccatcagacattgcttctcccatctgctctttcagctccgcattctcaaggcaaaggctcagcatggtgttcctgatgtgggacactgaggagaatcctgcttcctcaatttgagcctttagctccttcagttcctcctcagctttcctcttctcttctaagtgctggtggaactcagccctcaggtggagcatttcttcctgaagacacctgttactgtcccctcccatcggagaaggaggggaaaaagatgggttctgggtctccacagttgccagacttttctccaaagccaccttgacaagttgctggtgactatggtgtgcagcctcctcctcaatactgtcagtgaactcagtgcttgtatcttcggtgtcatcccctgcagctgcacctccaatggcggccagggtctccagcctgtttaagcgctccaagcttcttccaagaacttcttctagccgactgcgtaacacctgagccccttccagttccacctgcagagttcggtctctctcagagctctctggatgggcatggaacttcaccagactgctatagagctgtctctctgcttgtaaggcctcattgagccgactccgttcatctactagtccttctagcatcagcagcaactgttgtcttcggtttcctgaaatttcttgaccctgggattctactgaagcaactttttcccgaagaagtaagacttcctgggtcaggcgttccatagctggtatgtcttcaggatcaaccagttgcatttgcaggtcctttatgagatcttctttaatctgtatgttcctggtcagagactccatatcagcagcctgcacctgcagctcttcttcctgcacagccatcatggactgtagagcagaaagttccatctgactttctctttcttttttagccatgagttcaagttcctctttggcattactcagttctttttccagccctgcaactgtgtccaagtctcctaatgtggatctgggtatgctgacatcctctttggcagtcaatgaagtgctatcatctctggaaggtatctgcattgaaccttgatcagtctgttttccaagacggccagtgggggtaacttcagcttgttggttagagatgggtgcttgggacatcagggagtctctccctcctaaatattggcgcagggcctgtaattctgaatttctttccattaaggcttgcaccaacttctctgcagcagcttggctttcctgctccctggtgctcacagactgaagcaggccttgaatctccatttcatgttccagcacttgtttatttcgatcacttagaaggtcctgcagcatcctttcctttcgctgtagacgctggcacagctcctctgctatctcactctgccctggtccaagtttgcagagcagtgttgcactaagatcctccacttctttgttcctatcatgaagagacgtctgtaactgctgaatgatactctcttgttccttctgccaacggctaaatttggtttccatttcttctttcagccactggaggttttgacaggtagtagataactgttccacttccaggcctttggccctcaggagactctccatactttgcatagtagcttcattggaggagaggacatcgcgcagtctctctaagtcatgatctcgctctctcacagcaagacgaagctggcgcagttctttttctttctcttctagagcagagaatttttcatctatagcccgctccagagcaacagctttatcatgtattcgctggcgaagtttctcaagcaacatttcatttgcttcaagggttttgtctgagttatctcgatactgtaggagctcccgaaattcctgaagcaactgctccttgtgactcagactatggtttaggtgctggatgttttgttcctgggttcgaatctcattgtatttttcagcctcccaggcacgaagctgttggctcttattctgcaattcttcttgtagctgctgcaaggcttttcgcaattcctggttatgtttccaagaagcctctttctgctgttcactctcgtgtgctgcagcctctacaaattgcacacattgtttggcatcagccagttggcgctctttctgtcgtaccaccctctggagcttctgtatttcaagttggctgcagaataaagcactctgaagatcaagcagagctacctgttgctgagctggagaagtaccctctgagctgtgaagttgtccaagctggctttggtgcagcatttctcgaagctttgccattgtgtcattttgaccttcaattacctggtacaactcctcagtctcacgttccctgcttttcagagtttccttgaggttctgaattgtaccatcttgcttttgagacgactcctgagcacactttagttcatagctcatttcattaagtttctcttgaagaatcttgttggtggcctctgtttgctggattttttcctggagttctgccaagtgggaatcagatacagactgctgagttatagtggtctcatgtgaattcagcttttgttgtttcagcaactcttcagtcatgggctgcacttccatgctagttggctcctccaacagatgtagcagttgttgtttctcccgagatagctgttctacaagcctctcctgggcagccaggctctgattcagttcttcaattctcttgtccctctgggccagggcctcagtgtattggtcgggcttgacctggtctcctggtacatcttcccagtttttggtgactcccttcagtttctctgagagctccaggttacactccttctctgcttccaccagagctgccatccgcgcagcttcattctttgctagcctggattcctcctgcagaagctggatcttattctccaagagctcataaacatgctccgtctcctgctgtcgctcctcaaactggcgtcggagctcagcttcattctgactgttgagattctccacatcagccccgcttgtagatgtcctcccggctggcctcatacttctgttgcatgcgctcctccaggaagtagatgcgcagcttgaggctgaagttctccttcttcaggtcattgaggtgcttctcaaagtctcgaagagcctgggtctgtacctgagggggtttctcaaatgctctcaaggaatatgtctgcacaaacgggaccttttcaccacttctccagatctgtgactgcactggagggcctcgatctttagtgtcactaagaaaagctgctgtgtgactcgttctgggtaccatctccccatcatcctctgcaaaataatctctcgtccaggtctgctccattttccaggctctttccttagtctcaggacgctcctcacccgggaggggaagcagcctgggaaaatgagaagccttgcccacgaatctccagcgcaaaaggcagcagctttttcctccccagctcctttctgcgtcggcggcgaagagagagctctgctccctgcttttttagaaaatggatttgacgtggccgaacctgcggctagccgtgcgacccgcacaagggagggactgttctcagtaggaggctggactcagagcggcgcggcgcccggggctgtttcgtgagctggagccagcggctgcccgggccgcggtgcgcgcactctccaggctgagacacgactggct

SEQ ID NO: 8817 - RNA, 7676 nt, Homo sapiens
  source 1..7676: mol_type = other RNA
aagtgtgcagggcactggtgctgctccgaagctcatgaatacctttgctgcctagcacctctgtgccttgggcttcaaggccagggaagctgcacgctgatctcacaagagacactatctttttgaccagcagcttgccctccgcaatctgctgtcttagggcactgtagtcatcaatgtggccaatgacatggcggccatgcttattggcaaaggagccatcagtagcatcaccctctagcttgggaggggtcttcattactggagaagtatccaaacccaagccatttgctctgttgattatgggcgtttctgagccaggagtagaggaagcagagctggggaagaccagagctggggaattcataccaacatcccggactggaggggacacagctgaatcttggaggagcagctgcttgtttccagggtcagtgctggctgggaagttctggttaatggaggaggggctgaggctggctttgccagcaccgctctccagctgctgttgcagctgcagtcgcagacaattgttcccctgaatgctctgctccagctgccctctcagagctcgtacctctgccaccaggtggctcaggtcactgctcaaagggatttggtgacaggcatccaggctgtaagctttcagccccttcttggaattgccataaagtgcctcgtagatttgtagctctgactggagggactcaaagagctgctgtttctcttcacactgttgctgcaggagaaccagcttgtgctgcagtctggagtcgttttcctggagggaaagacgttcctccctgaaatgcaagacctcttgctgcttctccctcaagtcttccaaaagctgctgcctttccaccttctggtgctccagctccttttccagctcttgaaggtgggatcgagaggacagcagagcctccctcaggctttctgtttcctgggagtgctctctggaaacatgactcagttgagcctgaagtcttcgattgtcttccctgaggactctgttctcattgcagagctgaggtatggactccaggccctgactgtagaagttagaagtggatccccttccacgagcagtagaggtcagccggtgttccagttgctcccgtaggcggtcattgatgcagatggattcctccaggcgctggcgcaggttccggatttcaccaagatgctcttccagcaggtcagcccctgtgggtttggagttaagctggtacacagaggagcctgaggataggtccccagatacactccctttctgaggcctcatcacatcccacttgccactgctgcccaggtacccaggctctaggattcttcccagttctatggtgccccttggaggagagtgaggctgggcagagttgaggtagtaggaagagtcggcttccaagtcgttgctcagcaatgtagctgtggaagcaggaggaacagtgctggcactttctcccaactgcttctgcagcatctgtagctcctgctgagcctcagccaaggagaccactggtgtctcacagcagccaaggaggagagggccagtggggctgaaaggcaggaagctggatggagctgagggcaatggtgcctgaggaaggctagccagcttgggtatggagtgaaaatgaaagcctgaatgggcctggttggcctccttgggggtattctggggagttggcaagctgatggggttgctgttggattcggccttagccccctgagatgcactggttgatgatggtttagaagacaacacagcagaatgactcgaatgatggatggaatctgagtgactgggagaagctttcttctcttcatagtgtgtgtactcgctgactatgtccatgtcagagcaggcttccagttcatcagacaggaaagaggtgctgctgggagagcggtgggagtcagacaaggcatggctgctggagggtgtgagggaccgagcatccagcttggcctgcaggacttcaatcactttctccttctcctgcagctccctgctgagcctgagggccagtggctcaagtccagcttgatctttctcacttttatgatccttggtgctgagtttgctggtgagcctctctgtcagctggcttccctgggcgagttgctcccggaagctctgtcccaggtagtagtcaatgtcattgctccttaggagatcctcaaaagattttactgtatcttttgcatgccgggtgataagataacaaatacctctcccttctcgtattttttgccgtaggtaagacagttcccgggcctgatcctgaatcagggaatcatatttcccaggccacgaggctgatctcagctcctcagccagcttctcttctagtccattttttgggagctgggcctccagctgggatactctctggatgagactctccaggtcctttttggcctgaagccctggagagtagaaagccccagtgccatcagacagccacccctcatcctcatcagggacactatgaggtgaagacccctccaaggtgccaacagctctcagcttccggggtctttccagactagacgaataatcacttgtaactgagagggaccggacccggctcttgaggttttgaatgaccttgttggcattctgcagctgggccttcagatctttgatgtcctttcgtaggaccaagatgttttctgactttccatatacccggaactcttcctgcttccctagctggttctccaagggcttcctctcagaggaactagccagtgttgagccccggcgtccctgctcagagcacagcccctccatcaggaccatttccttgaggctgttgtgctcctcacactcaggactggtggtttcctcccgttcagcctcattctcgcttcggccacaagtctcatagcccaggtcctggaggtccacctggatctgcttgctgtcctgcttcaccaaggattcacctgtaagcataactctgtatttctccagctcgttagcctgagcaaagacagtggcttctgatagcagcagcttctcctggagatcttgatagcgttgtttgcattgtgacagctgggagcgcaggtgctgggtggaccctggtaggctaaacgctgactgaggcccagggtcacgaggctgggactggttatccaattggtgggcatccactgtgaaggtagccccaaggtcaaggctctggggtctggggaaaggcctcacagtcacattcccctcctcttggtgttggtgcttcccaggggaaccaaccagttctgtgtttattctttcaatggtgctggtcagatgcacaaggagctctggagtaagtttactattcccttccttgctactcagcacaagttgttctttgaggaggttgatgatattgtgggcattcttcagttttccctggagctttctgaactcagcctgaaggctactctcactcagaccctctttggttaccacagtctcaaccatcacctcgcccttctccttgtcttcctcgatctcccatccatcagacattgcttctcccatctgctctttcagctccgcattctcaaggcaaaggctcagcatggtgttcctgatgtgggacactgaggagaatcctgcttcctcaatttgagcctttagctccttcagttcctcctcagctttcctcttctcttctaagtgctggtggaactcagccctcaggtggagcatttcttcctgaagacacctgttactgtcccctcccatcggagaaggaggggaaaaagatgggttctgggtctccacagttgccagacttttctccaaagccaccttgacaagttgctggtgactatggtgtgcagcctcctcctcaatactgtcagtgaactcagtgcttgtatcttcggtgtcatcccctgcagctgcacctccaatggcggccagggtctccagcctgtttaagcgctccaagcttcttccaagaacttcttctagccgactgcgtaacacctgagccccttccagttccacctgcagagttcggtctctctcagagctctctggatgggcatggaacttcaccagactgctatagagctgtctctctgcttgtaaggcctcattgagccgactccgttcatctactagtccttctagcatcagcagcaactgttgtcttcggtttcctgaaatttcttgaccctgggattctactgaagcaactttttcccgaagaagtaagacttcctgggtcaggcgttccatagctggtatgtcttcaggatcaaccagttgcatttgcaggtcctttatgagatcttctttaatctgtatgttcctggtcagagactccatatcagcagcctgcacctgcagctcttcttcctgcacagccatcatggactgtagagcagaaagttccatctgactttctctttcttttttagccatgagttcaagttcctctttggcattactcagttctttttccagccctgcaactgtgtccaagtctcctaatgtggatctgggtatgctgacatcctctttggcagtcaatgaagtgctatcatctctggaaggtatctgcattgaaccttgatcagtctgttttccaagacggccagtgggggtaacttcagcttgttggttagagatgggtgcttgggacatcagggagtctctccctcctaaatattggcgcagggcctgtaattctgaatttctttccattaaggcttgcaccaacttctctgcagcagcttggctttcctgctccctggtgctcacagactgaagcaggccttgaatctccatttcatgttccagcacttgtttatttcgatcacttagaaggtcctgcagcatcctttcctttcgctgtagacgctggcacagctcctctgctatctcactctgccctggtccaagtttgcagagcagtgttgcactaagatcctccacttctttgttcctatcatgaagagacgtctgtaactgctgaatgatactctcttgttccttctgccaacggctaaatttggtttccatttcttctttcagccactggaggttttgacaggtagtagataactgttccacttccaggcctttggccctcaggagactctccatactttgcatagtagcttcattggaggagaggacatcgcgcagtctctctaagtcatgatctcgctctctcacagcaagacgaagctggcgcagttctttttctttctcttctagagcagagaatttttcatctatagcccgctccagagcaacagctttatcatgtattcgctggcgaagtttctcaagcaacatttcatttgcttcaagggttttgtctgagttatctcgatactgtaggagctcccgaaattcctgaagcaactgctccttgtgactcagactatggtttaggtgctggatgttttgttcctgggttcgaatctcattgtatttttcagcctcccaggcacgaagctgttggctcttattctgcaattcttcttgtagctgctgcaaggcttttcgcaattcctggttatgtttccaagaagcctctttctgctgttcactctcgtgtgctgcagcctctacaaattgcacacattgtttggcatcagccagttggcgctctttctgtcgtaccaccctctggagcttctgtatttcaagttggctgcagaataaagcactctgaagatcaagcagagctacctgttgctgagctggagaagtaccctctgagctgtgaagttgtccaagctggctttggtgcagcatttctcgaagctttgccattgtgtcattttgaccttcaattacctggtacaactcctcagtctcacgttccctgcttttcagagtttccttgaggttctgaattgtaccatcttgcttttgagacgactcctgagcacactttagttcatagctcatttcattaagtttctcttgaagaatcttgttggtggcctctgtttgctggattttttcctggagttctgccaagtgggaatcagatacagactgctgagttatagtggtctcatgtgaattcagcttttgttgtttcagcaactcttcagtcatgggctgcacttccatgctagttggctcctccaacagatgtagcagttgttgtttctcccgagatagctgttctacaagcctctcctgggcagccaggctctgattcagttcttcaattctcttgtccctctgggccagggcctcagtgtattggtcgggcttgacctggtctcctggtacatcttcccagtttttggtgactcccttcagtttctctgagagctccaggttacactccttctctgcttccaccagagctgccatccgcgcagcttcattctttgctagcctggattcctcctgcagaagctggatcttattctccaagagctcataaacatgctccgtctcctgctgtcgctcctcaaactggcgtcggagctcagcttcattctgactgttgagattctccacatcagccccgcttgtagatgtcctcccggctggcctcatacttctgttgcatgcgctcctccaggaagtagatgcgcagcttgaggctgaagttctccttcttcaggtcattgaggtgcttctcaaagtctcgaagagcctgggtctgtacctgagggggtttctcaaatgctctcaaggaatatgtctgcacaaacgggaccttttcaccacttctccagatctgtgactgcactggagggcctcgatctttagtgtcactaagaaaagcttctttccttcgttctgccaacttgccagaaggagcccaagaaaaagcacccagatgcttcagtcaacttcttagaattcttcttttttttatgttcagaaaagatggaaattcatttctgctgtgtgactcgttctgggtaccatctccccatcatcctctgcaaaataatctctcgtccaggtctgctccattttccaggctctttccttagtctcaggacgctcctcacccgggaggggaagcagcctgggaaaatgagaagccttgcccacgaatctccagcgcaaaaggcagcagctttttcctccccagctcctttctgcgtcggcggcgaagagagagctctgctccctgcttttttagaaaatggatttgacgtggccgaacctgcggctagccgtgcgacccgcacaagggagggactgttctcagtaggaggctggactcagagcggcgcggcgcccggggctgtttcgtgagctggagccagcggctgcccgggccgcggtgcgcgcactctccaggctgagacacgactggctggcacgagttgctcggcaccagctgagctgtcaaccgcgagcggaggcggggctcccgacaaccagtgtgctggggcagaatcggcccaggttacacgccccctgaaccaccctcgcgtctccccgacccctctctcgctggctcagatgaatgatgacggcagagggcagagagcttagaggacgcggtaccaagccccgtccctcgcccatcccaacgaaggtcttagaatacaatcaaccaactacaggaagaatttgtagaggaggttttcttgtgtgtctgcatcgccccacccacaggtaaccccagagccagagatggagtctaggaaggtttaggagcaatcccggctga

SEQ ID NO: 8818 - RNA, 7623 nt, Homo sapiens
  source 1..7623: mol_type = other RNA
aagtgtgcagggcactggtgctgctccgaagctcatgaatacctttgctgcctagcacctctgtgccttgggcttcaaggccagggaagctgcacgctgatctcacaagagacactatctttttgaccagcagcttgccctccgcaatctgctgtcttagggcactgtagtcatcaatgtggccaatgacatggcggccatgcttattggcaaaggagccatcagtagcatcaccctctagcttgggaggggtcttcattactggagaagtatccaaacccaagccatttgctctgttgattatgggcgtttctgagccaggagtagaggaagcagagctggggaagaccagagctggggaattcataccaacatcccggactggaggggacacagctgaatcttggaggagcagctgcttgtttccagggtcagtgctggctgggaagttctggttaatggaggaggggctgaggctggctttgccagcaccgctctccagctgctgttgcagctgcagtcgcagacaattgttcccctgaatgctctgctccagctgccctctcagagctcgtacctctgccaccaggtggctcaggtcactgctcaaagggatttggtgacaggcatccaggctgtaagctttcagccccttcttggaattgccataaagtgcctcgtagatttgtagctctgactggagggactcaaagagctgctgtttctcttcacactgttgctgcaggagaaccagcttgtgctgcagtctggagtcgttttcctggagggaaagacgttcctccctgaaatgcaagacctcttgctgcttctccctcaagtcttccaaaagctgctgcctttccaccttctggtgctccagctccttttccagctcttgaaggtgggatcgagaggacagcagagcctccctcaggctttctgtttcctgggagtgctctctggaaacatgactcagttgagcctgaagtcttcgattgtcttccctgaggactctgttctcattgcagagctgaggtatggactccaggccctgactgtagaagttagaagtggatccccttccacgagcagtagaggtcagccggtgttccagttgctcccgtaggcggtcattgatgcagatggattcctccaggcgctggcgcaggttccggatttcaccaagatgctcttccagcaggtcagcccctgtgggtttggagttaagctggtacacagaggagcctgaggataggtccccagatacactccctttctgaggcctcatcacatcccacttgccactgctgcccaggtacccaggctctaggattcttcccagttctatggtgccccttggaggagagtgaggctgggcagagttgaggtagtaggaagagtcggcttccaagtcgttgctcagcaatgtagctgtggaagcaggaggaacagtgctggcactttctcccaactgcttctgcagcatctgtagctcctgctgagcctcagccaaggagaccactggtgtctcacagcagccaaggaggagagggccagtggggctgaaaggcaggaagctggatggagctgagggcaatggtgcctgaggaaggctagccagcttgggtatggagtgaaaatgaaagcctgaatgggcctggttggcctccttgggggtattctggggagttggcaagctgatggggttgctgttggattcggccttagccccctgagatgcactggttgatgatggtttagaagacaacacagcagaatgactcgaatgatggatggaatctgagtgactgggagaagctttcttctcttcatagtgtgtgtactcgctgactatgtccatgtcagagcaggcttccagttcatcagacaggaaagaggtgctgctgggagagcggtgggagtcagacaaggcatggctgctggagggtgtgagggaccgagcatccagcttggcctgcaggacttcaatcactttctccttctcctgcagctccctgctgagcctgagggccagtggctcaagtccagcttgatctttctcacttttatgatccttggtgctgagtttgctggtgagcctctctgtcagctggcttccctgggcgagttgctcccggaagctctgtcccaggtagtagtcaatgtcattgctccttaggagatcctcaaaagattttactgtatcttttgcatgccgggtgataagataacaaatacctctcccttctcgtattttttgccgtaggtaagacagttcccgggcctgatcctgaatcagggaatcatatttcccaggccacgaggctgatctcagctcctcagccagcttctcttctagtccattttttgggagctgggcctccagctgggatactctctggatgagactctccaggtcctttttggcctgaagccctggagagtagaaagccccagtgccatcagacagccacccctcatcctcatcagggacactatgaggtgaagacccctccaaggtgccaacagctctcagcttccggggtctttccagactagacgaataatcacttgtaactgagagggaccggacccggctcttgaggttttgaatgaccttgttggcattctgcagctgggccttcagatctttgatgtcctttcgtaggaccaagatgttttctgactttccatatacccggaactcttcctgcttccctagctggttctccaagggcttcctctcagaggaactagccagtgttgagccccggcgtccctgctcagagcacagcccctccatcaggaccatttccttgaggctgttgtgctcctcacactcaggactggtggtttcctcccgttcagcctcattctcgcttcggccacaagtctcatagcccaggtcctggaggtccacctggatctgcttgctgtcctgcttcaccaaggattcacctgtaagcataactctgtatttctccagctcgttagcctgagcaaagacagtggcttctgatagcagcagcttctcctggagatcttgatagcgttgtttgcattgtgacagctgggagcgcaggtgctgggtggaccctggtaggctaaacgctgactgaggcccagggtcacgaggctgggactggttatccaattggtgggcatccactgtgaaggtagccccaaggtcaaggctctggggtctggggaaaggcctcacagtcacattcccctcctcttggtgttggtgcttcccaggggaaccaaccagttctgtgtttattctttcaatggtgctggtcagatgcacaaggagctctggagtaagtttactattcccttccttgctactcagcacaagttgttctttgaggaggttgatgatattgtgggcattcttcagttttccctggagctttctgaactcagcctgaaggctactctcactcagaccctctttggttaccacagtctcaaccatcacctcgcccttctccttgtcttcctcgatctcccatccatcagacattgcttctcccatctgctctttcagctccgcattctcaaggcaaaggctcagcatggtgttcctgatgtgggacactgaggagaatcctgcttcctcaatttgagcctttagctccttcagttcctcctcagctttcctcttctcttctaagtgctggtggaactcagccctcaggtggagcatttcttcctgaagacacctgttactgtcccctcccatcggagaaggaggggaaaaagatgggttctgggtctccacagttgccagacttttctccaaagccaccttgacaagttgctggtgactatggtgtgcagcctcctcctcaatactgtcagtgaactcagtgcttgtatcttcggtgtcatcccctgcagctgcacctccaatggcggccagggtctccagcctgtttaagcgctccaagcttcttccaagaacttcttctagccgactgcgtaacacctgagccccttccagttccacctgcagagttcggtctctctcagagctctctggatgggcatggaacttcaccagactgctatagagctgtctctctgcttgtaaggcctcattgagccgactccgttcatctactagtccttctagcatcagcagcaactgttgtcttcggtttcctgaaatttcttgaccctgggattctactgaagcaactttttcccgaagaagtaagacttcctgggtcaggcgttccatagctggtatgtcttcaggatcaaccagttgcatttgcaggtcctttatgagatcttctttaatctgtatgttcctggtcagagactccatatcagcagcctgcacctgcagctcttcttcctgcacagccatcatggactgtagagcagaaagttccatctgactttctctttcttttttagccatgagttcaagttcctctttggcattactcagttctttttccagccctgcaactgtgtccaagtctcctaatgtggatctgggtatgctgacatcctctttggcagtcaatgaagtgctatcatctctggaaggtatctgcattgaaccttgatcagtctgttttccaagacggccagtgggggtaacttcagcttgttggttagagatgggtgcttgggacatcagggagtctctccctcctaaatattggcgcagggcctgtaattctgaatttctttccattaaggcttgcaccaacttctctgcagcagcttggctttcctgctccctggtgctcacagactgaagcaggccttgaatctccatttcatgttccagcacttgtttatttcgatcacttagaaggtcctgcagcatcctttcctttcgctgtagacgctggcacagctcctctgctatctcactctgccctggtccaagtttgcagagcagtgttgcactaagatcctccacttctttgttcctatcatgaagagacgtctgtaactgctgaatgatactctcttgttccttctgccaacggctaaatttggtttccatttcttctttcagccactggaggttttgacaggtagtagataactgttccacttccaggcctttggccctcaggagactctccatactttgcatagtagcttcattggaggagaggacatcgcgcagtctctctaagtcatgatctcgctctctcacagcaagacgaagctggcgcagttctttttctttctcttctagagcagagaatttttcatctatagcccgctccagagcaacagctttatcatgtattcgctggcgaagtttctcaagcaacatttcatttgcttcaagggttttgtctgagttatctcgatactgtaggagctcccgaaattcctgaagcaactgctccttgtgactcagactatggtttaggtgctggatgttttgttcctgggttcgaatctcattgtatttttcagcctcccaggcacgaagctgttggctcttattctgcaattcttcttgtagctgctgcaaggcttttcgcaattcctggttatgtttccaagaagcctctttctgctgttcactctcgtgtgctgcagcctctacaaattgcacacattgtttggcatcagccagttggcgctctttctgtcgtaccaccctctggagcttctgtatttcaagttggctgcagaataaagcactctgaagatcaagcagagctacctgttgctgagctggagaagtaccctctgagctgtgaagttgtccaagctggctttggtgcagcatttctcgaagctttgccattgtgtcattttgaccttcaattacctggtacaactcctcagtctcacgttccctgcttttcagagtttccttgaggttctgaattgtaccatcttgcttttgagacgactcctgagcacactttagttcatagctcatttcattaagtttctcttgaagaatcttgttggtggcctctgtttgctggattttttcctggagttctgccaagtgggaatcagatacagactgctgagttatagtggtctcatgtgaattcagcttttgttgtttcagcaactcttcagtcatgggctggacccggagcggcaaataatcttcacagagatcatcccacagctcctgcaggtctgaaagctccaagggataactcacaggtgtcttgtaaaggggtttcaaagacctgttaaggaaaccggaactaactccatctgtcatgctagggccaggcttggctccaggtaggctggatttcactggaatcggaagcctgctccctcgggggctctggatgggcttataatcaagacctttaatcatgctaagagctaattccagcttgtgattacacccatgctgcggagcctgatcatctgaacaacagtcacactttccaagttcctttgcacttctctcagtctcctcatctttctgttgtggagggctagcctggacgcttgcatccaaagattccacagaggaaccaggcgtctcttcctccatgctttctccatctgggggtacctttgtgcttgctaagtcgggtggcccaacctcagacaacgctggttcttcagtgcaaatgctggtcgaccacctgctagaagggccgcaggagatacttctggccacctttcgaggtaccttacaaatggcttcatagtcagaatcagcaacccgcaaagcggcacaaccacggcatctcctgggtcggtttccagggccttctgaaccatggcagctgtgtggctcctggatctgatcctcattctccacccagcactcaaaccctgaataggcgaagtcctcctggagcagtgcagagtatctcgcatcgggtaagacggacatgtcaaccgtcccattccccgccttgatctccgcgccagagtcatcgttattcttccgatacatactggcaatgcagaacttgaggcgatccttctccagtagcagcttttgcaagcgctcaatagaaagcgcttcaatccgggcaataactgtgtcgaatcgatagattcgatcaagcatgaaagcacacttgctgcaagcgaactcggctttgccatcgcgggggacatccttgcccaagacgtgcgaaagcagaacctggagattgagcttggacgccgtgtggaagatccagcgccgctggtttccacacagctctcgggcacagatcctgcaaatctccttcatcttccctcctagcgggtggcaagcttcccgaggcggcggcggcggcggctactgggtgaccactcaatggctcttcgccgcgctctgtctcccgcctcggtggtctccggtcagcatggcacagcccagtggggtccccactctgcaggggcgcgcccctgccccgcgcgccgactccgggtaccagagccgtcagccccgcccctcgggcagggggcgggcgtggaaacgcctaagaggatgctgagtgacagaggcgcaggccgcgctccgaccctgccatgtctctccccagctgtctctcccgccagccgccgcgtcctcaacgtcctccccttttagcagactgggctcccggagcagcagcggccggccgcgcagacgcaaagcctcggggatggaggatc

SEQ ID NO: 8819 - RNA, 7290 nt, Homo sapiens
  source 1..7290: mol_type = other RNA
aagtgtgcagggcactggtgctgctccgaagctcatgaatacctttgctgcctagcacctctgtgccttgggcttcaaggccagggaagctgcacgctgatctcacaagagacactatctttttgaccagcagcttgccctccgcaatctgctgtcttagggcactgtagtcatcaatgtggccaatgacatggcggccatgcttattggcaaaggagccatcagtagcatcaccctctagcttgggaggggtcttcattactggagaagtatccaaacccaagccatttgctctgttgattatgggcgtttctgagccaggagtagaggaagcagagctggggaagaccagagctggggaattcataccaacatcccggactggaggggacacagctgaatcttggaggagcagctgcttgtttccagggtcagtgctggctgggaagttctggttaatggaggaggggctgaggctggctttgccagcaccgctctccagctgctgttgcagctgcagtcgcagacaattgttcccctgaatgctctgctccagctgccctctcagagctcgtacctctgccaccaggtggctcaggtcactgctcaaagggatttggtgacaggcatccaggctgtaagctttcagccccttcttggaattgccataaagtgcctcgtagatttgtagctctgactggagggactcaaagagctgctgtttctcttcacactgttgctgcaggagaaccagcttgtgctgcagtctggagtcgttttcctggagggaaagacgttcctccctgaaatgcaagacctcttgctgcttctccctcaagtcttccaaaagctgctgcctttccaccttctggtgctccagctccttttccagctcttgaaggtgggatcgagaggacagcagagcctccctcaggctttctgtttcctgggagtgctctctggaaacatgactcagttgagcctgaagtcttcgattgtcttccctgaggactctgttctcattgcagagctgaggtatggactccaggccctgactgtagaagttagaagtggatccccttccacgagcagtagaggtcagccggtgttccagttgctcccgtaggcggtcattgatgcagatggattcctccaggcgctggcgcaggttccggatttcaccaagatgctcttccagcaggtcagcccctgtgggtttggagttaagctggtacacagaggagcctgaggataggtccccagatacactccctttctgaggcctcatcacatcccacttgccactgctgcccaggtacccaggctctaggattcttcccagttctatggtgccccttggaggagagtgaggctgggcagagttgaggtagtaggaagagtcggcttccaagtcgttgctcagcaatgtagctgtggaagcaggaggaacagtgctggcactttctcccaactgcttctgcagcatctgtagctcctgctgagcctcagccaaggagaccactggtgtctcacagcagccaaggaggagagggccagtggggctgaaaggcaggaagctggatggagctgagggcaatggtgcctgaggaaggctagccagcttgggtatggagtgaaaatgaaagcctgaatgggcctggttggcctccttgggggtattctggggagttggcaagctgatggggttgctgttggattcggccttagccccctgagatgcactggttgatgatggtttagaagacaacacagcagaatgactcgaatgatggatggaatctgagtgactgggagaagctttcttctcttcatagtgtgtgtactcgctgactatgtccatgtcagagcaggcttccagttcatcagacaggaaagaggtgctgctgggagagcggtgggagtcagacaaggcatggctgctggagggtgtgagggaccgagcatccagcttggcctgcaggacttcaatcactttctccttctcctgcagctccctgctgagcctgagggccagtggctcaagtccagcttgatctttctcacttttatgatccttggtgctgagtttgctggtgagcctctctgtcagctggcttccctgggcgagttgctcccggaagctctgtcccaggtagtagtcaatgtcattgctccttaggagatcctcaaaagattttactgtatcttttgcatgccgggtgataagataacaaatacctctcccttctcgtattttttgccgtaggtaagacagttcccgggcctgatcctgaatcagggaatcatatttcccaggccacgaggctgatctcagctcctcagccagcttctcttctagtccattttttgggagctgggcctccagctgggatactctctggatgagactctccaggtcctttttggcctgaagccctggagagtagaaagccccagtgccatcagacagccacccctcatcctcatcagggacactatgaggtgaagacccctccaaggtgccaacagctctcagcttccggggtctttccagactagacgaataatcacttgtaactgagagggaccggacccggctcttgaggttttgaatgaccttgttggcattctgcagctgggccttcagatctttgatgtcctttcgtaggaccaagatgttttctgactttccatatacccggaactcttcctgcttccctagctggttctccaagggcttcctctcagaggaactagccagtgttgagccccggcgtccctgctcagagcacagcccctccatcaggaccatttccttgaggctgttgtgctcctcacactcaggactggtggtttcctcccgttcagcctcattctcgcttcggccacaagtctcatagcccaggtcctggaggtccacctggatctgcttgctgtcctgcttcaccaaggattcactaagcataactctgtatttctccagctcgttagcctgagcaaagacagtggcttctgatagcagcagcttctcctggagatcttgatagcgttgtttgcattgtgacagctgggagcgcaggtgctgggtggaccctggtaggctaaacgctgactgaggcccagggtcacgaggctgggactggttatccaactcgcccttctccttgtcttcctcgatctcccatccatcagacattgcttctcccatctgctctttcagctccgcattctcaaggcaaaggctcagcatggtgttcctgatgtgggacactgaggagaatcctgcttcctcaatttgagcctttagctccttcagttcctcctcagctttcctcttctcttctaagtgctggtggaactcagccctcaggtggagcatttcttcctgaagacacctgttactgtcccctcccatcggagaaggaggggaaaaagatgggttctgggtctccacagttgccagacttttctccaaagccaccttgacaagttgctggtgactatggtgtgcagcctcctcctcaatactgtcagtgaactcagtgcttgtatcttcggtgtcatcccctgcagctgcacctccaatggcggccagggtctccagcctgtttaagcgctccaagcttcttccaagaacttcttctagccgactgcgtaacacctgagccccttccagttccacctgcagagttcggtctctctcagagctctctggatgggcatggaacttcaccagactgctatagagctgtctctctgcttgtaaggcctcattgagccgactccgttcatctactagtccttctagcatcagcagcaactgttgtcttcggtttcctgaaatttcttgaccctgggattctactgaagcaactttttcccgaagaagtaagacttcctgggtcaggcgttccatagctggtatgtcttcaggatcaaccagttgcatttgcaggtcctttatgagatcttctttaatctgtatgttcctggtcagagactccatatcagcagcctgcacctgcagctcttcttcctgcacagccatcatggactgtagagcagaaagttccatctgactttctctttcttttttagccatgagttcaagttcctctttggcattactcagttctttttccagccctgcaactgtgtccaagtctcctaatgtggatctgggtatgctgacatcctctttggcagtcaatgaagtgctatcatctctggaaggtatctgcattgaaccttgatcagtctgttttccaagacggccagtgggggtaacttcagcttgttggttagagatgggtgcttgggacatcagggagtctctccctcctaaatattggcgcagggcctgtaattctgaatttctttccattaaggcttgcaccaacttctctgcagcagcttggctttcctgctccctggtgctcacagactgaagcaggccttgaatctccatttcatgttccagcacttgtttatttcgatcacttagaaggtcctgcagcatcctttcctttcgctgtagacgctggcacagctcctctgctatctcactctgccctggtccaagtttgcagagcagtgttgcactaagatcctccacttctttgttcctatcatgaagagacgtctgtaactgctgaatgatactctcttgttccttctgccaacggctaaatttggtttccatttcttctttcagccactggaggttttgacaggtagtagataactgttccacttccaggcctttggccctcaggagactctccatactttgcatagtagcttcattggaggagaggacatcgcgcagtctctctaagtcatgatctcgctctctcacagcaagacgaagctggcgcagttctttttctttctcttctagagcagagaatttttcatctatagcccgctccagagcaacagctttatcatgtattcgctggcgaagtttctcaagcaacatttcatttgcttcaagggttttgtctgagttatctcgatactgtaggagctcccgaaattcctgaagcaactgctccttgtgactcagactatggtttaggtgctggatgttttgttcctgggttcgaatctcattgtatttttcagcctcccaggcacgaagctgttggctcttattctgcaattcttcttgtagctgctgcaaggcttttcgcaattcctggttatgtttccaagaagcctctttctgctgttcactctcgtgtgctgcagcctctacaaattgcacacattgtttggcatcagccagttggcgctctttctgtcgtaccaccctctggagcttctgtatttcaagttggctgcagaataaagcactctgaagatcaagcagagctacctgttgctgagctggagaagtaccctctgagctgtgaagttgtccaagctggctttggtgcagcatttctcgaagctttgccattgtgtcattttgaccttcaattacctggtacaactcctcagtctcacgttccctgcttttcagagtttccttgaggttctgaattgtaccatcttgcttttgagacgactcctgagcacactttagttcatagctcatttcattaagtttctcttgaagaatcttgttggtggcctctgtttgctggattttttcctggagttctgccaagtgggaatcagatacagactgctgagttatagtggtctcatgtgaattcagcttttgttgtttcagcaactcttcagtcatgggctggacccggagcggcaaataatcttcacagagatcatcccacagctcctgcaggtctgaaagctccaagggataactcacaggtgtcttgtaaaggggtttcaaagacctgttaaggaaaccggaactaactccatctgtcatgctagggccaggcttggctccaggtaggctggatttcactggaatcggaagcctgctccctcgggggctctggatgggcttataatcaagacctttaatcatgctaagagctaattccagcttgtgattacacccatgctgcggagcctgatcatctgaacaacagtcacactttccaagttcctttgcacttctctcagtctcctcatctttctgttgtggagggctagcctggacgcttgcatccaaagattccacagaggaaccaggcgtctcttcctccatgctttctccatctgggggtacctttgtgcttgctaagtcgggtggcccaacctcagacaacgctggttcttcagtgcaaatgctggtcgaccacctgctagaagggccgcaggagatacttctggccacctttcgaggtaccttacaaatggcttcatagtcagaatcagcaacccgcaaagcggcacaaccacggcatctcctgggtcggtttccagggccttctgaaccatggcagctgtgtggctcctggatctgatcctcattctccacccagcactcaaaccctgaataggcgaagtcctcctggagcagtgcagagtatctcgcatcgggtaagacggacatgtcaaccgtcccattccccgccttgatctccgcgccagagtcatcgttattcttccgatacatactggcaatgcagaacttgaggcgatccttctccagtagcagcttttgcaagcgctcaatagaaagcgcttcaatccgggcaataactgtgtcgaatcgatagattcgatcaagcatgaaagcacacttgctgcaagcgaactcggctttgccatcgcgggggacatccttgcccaagacgtgcgaaagcagaacctggagattgagcttggacgccgtgtggaagatccagcgccgctggtttccacacagctctcgggcacagatcctgcaaatctccttcatcttccctcctagcgggtggcaagcttcccgaggcggcggcggcggcggctactgggtgaccactcaatggctcttcgccgcgctctgtctcccgcctcggtggtctccggtcagcatggcacagcccagtggggtccccactctgcaggggcgcgcccctgccccgcgcgccgactccgggtaccagagccgtcagccccgcccctcgggcagggggcgggcgtggaaacgcctaagaggatgctgagtgacagaggcgcaggccgcgctccgaccctgccatgtctctccccagctgtctctcccgccagccgccgcgtcctcaacgtcctccccttttagcagactgggctcccggagcagcagcggccggccgcgcagacgcaaagcctcggggatggaggatc

SEQ ID NO: 8820 - RNA, 6918 nt, Homo sapiens
  source 1..6918: mol_type = other RNA
aagtgtgcagggcactggtgctgctccgaagctcatgaatacctttgctgcctagcacctctgtgccttgggcttcaaggccagggaagctgcacgctgatctcacaagagacactatctttttgaccagcagcttgccctccgcaatctgctgtcttagggcactgtagtcatcaatgtggccaatgacatggcggccatgcttattggcaaaggagccatcagtagcatcaccctctagcttgggaggggtcttcattactggagaagtatccaaacccaagccatttgctctgttgattatgggcgtttctgagccaggagtagaggaagcagagctggggaagaccagagctggggaattcataccaacatcccggactggaggggacacagctgaatcttggaggagcagctgcttgtttccagggtcagtgctggctgggaagttctggttaatggaggaggggctgaggctggctttgccagcaccgctctccagctgctgttgcagctgcagtcgcagacaattgttcccctgaatgctctgctccagctgccctctcagagctcgtacctctgccaccaggtggctcaggtcactgctcaaagggatttggtgacaggcatccaggctgtaagctttcagccccttcttggaattgccataaagtgcctcgtagatttgtagctctgactggagggactcaaagagctgctgtttctcttcacactgttgctgcaggagaaccagcttgtgctgcagtctggagtcgttttcctggagggaaagacgttcctccctgaaatgcaagacctcttgctgcttctccctcaagtcttccaaaagctgctgcctttccaccttctggtgctccagctccttttccagctcttgaaggtgggatcgagaggacagcagagcctccctcaggctttctgtttcctgggagtgctctctggaaacatgactcagttgagcctgaagtcttcgattgtcttccctgaggactctgttctcattgcagagctgaggtatggactccaggccctgactgtagaagttagaagtggatccccttccacgagcagtagaggtcagccggtgttccagttgctcccgtaggcggtcattgatgcagatggattcctccaggcgctggcgcaggttccggatttcaccaagatgctcttccagcaggtcagcccctgtgggtttggagttaagctggtacacagaggagcctgaggataggtccccagatacactccctttctgaggcctcatcacatcccacttgccactgctgcccaggtacccaggctctaggattcttcccagttctatggtgccccttggaggagagtgaggctgggcagagttgaggtagtaggaagagtcggcttccaagtcgttgctcagcaatgtagctgtggaagcaggaggaacagtgctggcactttctcccaactgcttctgcagcatctgtagctcctgctgagcctcagccaaggagaccactggtgtctcacagcagccaaggaggagagggccagtggggctgaaaggcaggaagctggatggagctgagggcaatggtgcctgaggaaggctagccagcttgggtatggagtgaaaatgaaagcctgaatgggcctggttggcctccttgggggtattctggggagttggcaagctgatggggttgctgttggattcggccttagccccctgagatgcactggttgatgatggtttagaagacaacacagcagaatgactcgaatgatggatggaatctgagtgactgggagaagctttcttctcttcatagtgtgtgtactcgctgactatgtccatgtcagagcaggcttccagttcatcagacaggaaagaggtgctgctgggagagcggtgggagtcagacaaggcatggctgctggagggtgtgagggaccgagcatccagcttggcctgcaggacttcaatcactttctccttctcctgcagctccctgctgagcctgagggccagtggctcaagtccagcttgatctttctcacttttatgatccttggtgctgagtttgctggtgagcctctctgtcagctggcttccctgggcgagttgctcccggaagctctgtcccaggtagtagtcaatgtcattgctccttaggagatcctcaaaagattttactgtatcttttgcatgccgggtgataagataacaaatacctctcccttctcgtattttttgccgtaggtaagacagttcccgggcctgatcctgaatcagggaatcatatttcccaggccacgaggctgatctcagctcctcagccagcttctcttctagtccattttttgggagctgggcctccagctgggatactctctggatgagactctccaggtcctttttggcctgaagccctggagagtagaaagccccagtgccatcagacagccacccctcatcctcatcagggacactatgaggtgaagacccctccaaggtgccaacagctctcagcttccggggtctttccagactagacgaataatcacttgtaactgagagggaccggacccggctcttgaggttttgaatgaccttgttggcattctgcagctgggccttcagatctttgatgtcctttcgtaggaccaagatgttttctgactttccatatacccggaactcttcctgcttccctagctggttctccaagggcttcctctcagaggaactagccagtgttgagccccggcgtccctgctcagagcacagcccctccatcaggaccatttccttgaggctgttgtgctcctcacactcaggactggtggtttcctcccgttcagcctcattctcgcttcggccacaagtctcatagcccaggtcctggaggtccacctggatctgcttgctgtcctgcttcaccaaggattcactaagcataactctgtatttctccagctcgttagcctgagcaaagacagtggcttctgatagcagcagcttctcctggagatcttgatagcgttgtttgcattgtgacagctgggagcgcaggtgctgggtggaccctggtaggctaaacgctgactgaggcccagggtcacgaggctgggactggttatccaattggtgggcatccactgtgaaggtagccccaaggtcaaggctctggggtctggggaaaggcctcacagtcacattcccctcctcttggtgttggtgcttcccaggggaaccaaccagttctgtgtttattctttcaatggtgctggtcagatgcacaaggagctctggagtaagtttactattcccttccttgctactcagcacaagttgttctttgaggaggttgatgatattgtgggcattcttcagttttccctggagctttctgaactcagcctgaaggctactctcactcagaccctctttggttaccacagtctcaaccatcacctcgcccttctccttgtcttcctcgatctcccatccatcagacattgcttctcccatctgctctttcagctccgcattctcaaggcaaaggctcagcatggtgttcctgatgtgggacactgaggagaatcctgcttcctcaatttgagcctttagctccttcagttcctcctcagctttcctcttctcttctaagtgctggtggaactcagccctcaggtggagcatttcttcctgaagacacctgttactgtcccctcccatcggagaaggaggggaaaaagatgggttctgggtctccacagttgccagacttttctccaaagccaccttgacaagttgctggtgactatggtgtgcagcctcctcctcaatactgtcagtgaactcagtgcttgtatcttcggtgtcatcccctgcagctgcacctccaatggcggccagggtctccagcctgtttaagcgctccaagcttcttccaagaacttcttctagccgactgcgtaacacctgagccccttccagttccacctgcagagttcggtctctctcagagctctctggatgggcatggaacttcaccagactgctatagagctgtctctctgcttgtaaggcctcattgagccgactccgttcatctactagtccttctagcatcagcagcaactgttgtcttcggtttcctgaaatttcttgaccctgggattctactgaagcaactttttcccgaagaagtaagacttcctgggtcaggcgttccatagctggtatgtcttcaggatcaaccagttgcatttgcaggtcctttatgagatcttctttaatctgtatgttcctggtcagagactccatatcagcagcctgcacctgcagctcttcttcctgcacagccatcatggactgtagagcagaaagttccatctgactttctctttcttttttagccatgagttcaagttcctctttggcattactcagttctttttccagccctgcaactgtgtccaagtctcctaatgtggatctgggtatgctgacatcctctttggcagtcaatgaagtgctatcatctctggaaggtatctgcattgaaccttgatcagtctgttttccaagacggccagtgggggtaacttcagcttgttggttagagatgggtgcttgggacatcagggagtctctccctcctaaatattggcgcagggcctgtaattctgaatttctttccattaaggcttgcaccaacttctctgcagcagcttggctttcctgctccctggtgctcacagactgaagcaggccttgaatctccatttcatgttccagcacttgtttatttcgatcacttagaaggtcctgcagcatcctttcctttcgctgtagacgctggcacagctcctctgctatctcactctgccctggtccaagtttgcagagcagtgttgcactaagatcctccacttctttgttcctatcatgaagagacgtctgtaactgctgaatgatactctcttgttccttctgccaacggctaaatttggtttccatttcttctttcagccactggaggttttgacaggtagtagataactgttccacttccaggcctttggccctcaggagactctccatactttgcatagtagcttcattggaggagaggacatcgcgcagtctctctaagtcatgatctcgctctctcacagcaagacgaagctggcgcagttctttttctttctcttctagagcagagaatttttcatctatagcccgctccagagcaacagctttatcatgtattcgctggcgaagtttctcaagcaacatttcatttgcttcaagggttttgtctgagttatctcgatactgtaggagctcccgaaattcctgaagcaactgctccttgtgactcagactatggtttaggtgctggatgttttgttcctgggttcgaatctcattgtatttttcagcctcccaggcacgaagctgttggctcttattctgcaattcttcttgtagctgctgcaaggcttttcgcaattcctggttatgtttccaagaagcctctttctgctgttcactctcgtgtgctgcagcctctacaaattgcacacattgtttggcatcagccagttggcgctctttctgtcgtaccaccctctggagcttctgtatttcaagttggctgcagaataaagcactctgaagatcaagcagagctacctgttgctgagctggagaagtaccctctgagctgtgaagttgtccaagctggctttggtgcagcatttctcgaagctttgccattgtgtcattttgaccttcaattacctggtacaactcctcagtctcacgttccctgcttttcagagtttccttgaggttctgaattgtaccatcttgcttttgagacgactcctgagcacactttagttcatagctcatttcattaagtttctcttgaagaatcttgttggtggcctctgtttgctggattttttcctggagttctgccaagtgggaatcagatacagactgctgagttatagtggtctcatgtgaattcagcttttgttgtttcagcaactcttcagtcatgggctgcacttccatgctagttggctcctccaacagatgtagcagttgttgtttctcccgagatagctgttctacaagcctctcctgggcagccaggctctgattcagttcttcaattctcttgtccctctgggccagggcctcagtgtattggtcgggcttgacctggtctcctggtacatcttcccagtttttggtgactcccttcagtttctctgagagctccaggttacactccttctctgcttccaccagagctgccatccgcgcagcttcattctttgctagcctggattcctcctgcagaagctggatcttattctccaagagctcataaacatgctccgtctcctgctgtcgctcctcaaactggcgtcggagctcagcttcattctgactgttgagattctccacatcagcccatgttttatccagatgctgtttcttgtcctggagttctcgtttcaagctctccacttcaaccttcagctcaatgttccgcttgtagatgtcctcccggctggcctcatacttctgttgcatgcgctcctccaggaagtagatgcgcagcttgaggctgaagttctccttcttcaggtcattgaggtgctgggacagagtgcgatatccattagacatgatgggcaacccatggggaggagcgtgcccgattgccccctcaacccaggaacatggtgcagctgcaccgcagcatgaagccagccggctgggacgctgctgaggctgcggaccgagaggctggggctacggcgacatggcccctattgctggagctctctccgggactcgggactgggctcactgctctgggt

SEQ ID NO: 8821 - RNA, 7442 nt, Homo sapiens
  source 1..7442: mol_type = other RNA
aagtgtgcagggcactggtgctgctccgaagctcatgaatacctttgctgcctagcacctctgtgccttgggcttcaaggccagggaagctgcacgctgatctcacaagagacactatctttttgaccagcagcttgccctccgcaatctgctgtcttagggcactgtagtcatcaatgtggccaatgacatggcggccatgcttattggcaaaggagccatcagtagcatcaccctctagcttgggaggggtcttcattactggagaagtatccaaacccaagccatttgctctgttgattatgggcgtttctgagccaggagtagaggaagcagagctggggaagaccagagctggggaattcataccaacatcccggactggaggggacacagctgaatcttggaggagcagctgcttgtttccagggtcagtgctggctgggaagttctggttaatggaggaggggctgaggctggctttgccagcaccgctctccagctgctgttgcagctgcagtcgcagacaattgttcccctgaatgctctgctccagctgccctctcagagctcgtacctctgccaccaggtggctcaggtcactgctcaaagggatttggtgacaggcatccaggctgtaagctttcagccccttcttggaattgccataaagtgcctcgtagatttgtagctctgactggagggactcaaagagctgctgtttctcttcacactgttgctgcaggagaaccagcttgtgctgcagtctggagtcgttttcctggagggaaagacgttcctccctgaaatgcaagacctcttgctgcttctccctcaagtcttccaaaagctgctgcctttccaccttctggtgctccagctccttttccagctcttgaaggtgggatcgagaggacagcagagcctccctcaggctttctgtttcctgggagtgctctctggaaacatgactcagttgagcctgaagtcttcgattgtcttccctgaggactctgttctcattgcagagctgaggtatggactccaggccctgactgtagaagttagaagtggatccccttccacgagcagtagaggtcagccggtgttccagttgctcccgtaggcggtcattgatgcagatggattcctccaggcgctggcgcaggttccggatttcaccaagatgctcttccagcaggtcagcccctgtgggtttggagttaagctggtacacagaggagcctgaggataggtccccagatacactccctttctgaggcctcatcacatcccacttgccactgctgcccaggtacccaggctctaggattcttcccagttctatggtgccccttggaggagagtgaggctgggcagagttgaggtagtaggaagagtcggcttccaagtcgttgctcagcaatgtagctgtggaagcaggaggaacagtgctggcactttctcccaactgcttctgcagcatctgtagctcctgctgagcctcagccaaggagaccactggtgtctcacagcagccaaggaggagagggccagtggggctgaaaggcaggaagctggatggagctgagggcaatggtgcctgaggaaggctagccagcttgggtatggagtgaaaatgaaagcctgaatgggcctggttggcctccttgggggtattctggggagttggcaagctgatggggttgctgttggattcggccttagccccctgagatgcactggttgatgatggtttagaagacaacacagcagaatgactcgaatgatggatggaatctgagtgactgggagaagctttcttctcttcatagtgtgtgtactcgctgactatgtccatgtcagagcaggcttccagttcatcagacaggaaagaggtgctgctgggagagcggtgggagtcagacaaggcatggctgctggagggtgtgagggaccgagcatccagcttggcctgcaggacttcaatcactttctccttctcctgcagctccctgctgagcctgagggccagtggctcaagtccagcttgatctttctcacttttatgatccttggtgctgagtttgctggtgagcctctctgtcagctggcttccctgggcgagttgctcccggaagctctgtcccaggtagtagtcaatgtcattgctccttaggagatcctcaaaagattttactgtatcttttgcatgccgggtgataagataacaaatacctctcccttctcgtattttttgccgtaggtaagacagttcccgggcctgatcctgaatcagggaatcatatttcccaggccacgaggctgatctcagctcctcagccagcttctcttctagtccattttttgggagctgggcctccagctgggatactctctggatgagactctccaggtcctttttggcctgaagccctggagagtagaaagccccagtgccatcagacagccacccctcatcctcatcagggacactatgaggtgaagacccctccaaggtgccaacagctctcagcttccggggtctttccagactagacgaataatcacttgtaactgagagggaccggacccggctcttgaggttttgaatgaccttgttggcattctgcagctgggccttcagatctttgatgtcctttcgtaggaccaagatgttttctgactttccatatacccggaactcttcctgcttccctagctggttctccaagggcttcctctcagaggaactagccagtgttgagccccggcgtccctgctcagagcacagcccctccatcaggaccatttccttgaggctgttgtgctcctcacactcaggactggtggtttcctcccgttcagcctcattctcgcttcggccacaagtctcatagcccaggtcctggaggtccacctggatctgcttgctgtcctgcttcaccaaggattcactaagcataactctgtatttctccagctcgttagcctgagcaaagacagtggcttctgatagcagcagcttctcctggagatcttgatagcgttgtttgcattgtgacagctgggagcgcaggtgctgggtggaccctggtaggctaaacgctgactgaggcccagggtcacgaggctgggactggttatccaattggtgggcatccactgtgaaggtagccccaaggtcaaggctctggggtctggggaaaggcctcacagtcacattcccctcctcttggtgttggtgcttcccaggggaaccaaccagttctgtgtttattctttcaatggtgctggtcagatgcacaaggagctctggagtaagtttactattcccttccttgctactcagcacaagttgttctttgaggaggttgatgatattgtgggcattcttcagttttccctggagctttctgaactcagcctgaaggctactctcactcagaccctctttggttaccacagtctcaaccatcacctcgcccttctccttgtcttcctcgatctcccatccatcagacattgcttctcccatctgctctttcagctccgcattctcaaggcaaaggctcagcatggtgttcctgatgtgggacactgaggagaatcctgcttcctcaatttgagcctttagctccttcagttcctcctcagctttcctcttctcttctaagtgctggtggaactcagccctcaggtggagcatttcttcctgaagacacctgttactgtcccctcccatcggagaaggaggggaaaaagatgggttctgggtctccacagttgccagacttttctccaaagccaccttgacaagttgctggtgactatggtgtgcagcctcctcctcaatactgtcagtgaactcagtgcttgtatcttcggtgtcatcccctgcagctgcacctccaatggcggccagggtctccagcctgtttaagcgctccaagcttcttccaagaacttcttctagccgactgcgtaacacctgagccccttccagttccacctgcagagttcggtctctctcagagctctctggatgggcatggaacttcaccagactgctatagagctgtctctctgcttgtaaggcctcattgagccgactccgttcatctactagtccttctagcatcagcagcaactgttgtcttcggtttcctgaaatttcttgaccctgggattctactgaagcaactttttcccgaagaagtaagacttcctgggtcaggcgttccatagctggtatgtcttcaggatcaaccagttgcatttgcaggtcctttatgagatcttctttaatctgtatgttcctggtcagagactccatatcagcagcctgcacctgcagctcttcttcctgcacagccatcatggactgtagagcagaaagttccatctgactttctctttcttttttagccatgagttcaagttcctctttggcattactcagttctttttccagccctgcaactgtgtccaagtctcctaatgtggatctgggtatgctgacatcctctttggcagtcaatgaagtgctatcatctctggaaggtatctgcattgaaccttgatcagtctgttttccaagacggccagtgggggtaacttcagcttgttggttagagatgggtgcttgggacatcagggagtctctccctcctaaatattggcgcagggcctgtaattctgaatttctttccattaaggcttgcaccaacttctctgcagcagcttggctttcctgctccctggtgctcacagactgaagcaggccttgaatctccatttcatgttccagcacttgtttatttcgatcacttagaaggtcctgcagcatcctttcctttcgctgtagacgctggcacagctcctctgctatctcactctgccctggtccaagtttgcagagcagtgttgcactaagatcctccacttctttgttcctatcatgaagagacgtctgtaactgctgaatgatactctcttgttccttctgccaacggctaaatttggtttccatttcttctttcagccactggaggttttgacaggtagtagataactgttccacttccaggcctttggccctcaggagactctccatactttgcatagtagcttcattggaggagaggacatcgcgcagtctctctaagtcatgatctcgctctctcacagcaagacgaagctggcgcagttctttttctttctcttctagagcagagaatttttcatctatagcccgctccagagcaacagctttatcatgtattcgctggcgaagtttctcaagcaacatttcatttgcttcaagggttttgtctgagttatctcgatactgtaggagctcccgaaattcctgaagcaactgctccttgtgactcagactatggtttaggtgctggatgttttgttcctgggttcgaatctcattgtatttttcagcctcccaggcacgaagctgttggctcttattctgcaattcttcttgtagctgctgcaaggcttttcgcaattcctggttatgtttccaagaagcctctttctgctgttcactctcgtgtgctgcagcctctacaaattgcacacattgtttggcatcagccagttggcgctctttctgtcgtaccaccctctggagcttctgtatttcaagttggctgcagaataaagcactctgaagatcaagcagagctacctgttgctgagctggagaagtaccctctgagctgtgaagttgtccaagctggctttggtgcagcatttctcgaagctttgccattgtgtcattttgaccttcaattacctggtacaactcctcagtctcacgttccctgcttttcagagtttccttgaggttctgaattgtaccatcttgcttttgagacgactcctgagcacactttagttcatagctcatttcattaagtttctcttgaagaatcttgttggtggcctctgtttgctggattttttcctggagttctgccaagtgggaatcagatacagactgctgagttatagtggtctcatgtgaattcagcttttgttgtttcagcaactcttcagtcatgggctgcacttccatgctagttggctcctccaacagatgtagcagttgttgtttctcccgagatagctgttctacaagcctctcctgggcagccaggctctgattcagttcttcaattctcttgtccctctgggccagggcctcagtgtattggtcgggcttgacctggtctcctggtacatcttcccagtttttggtgactcccttcagtttctctgagagctccaggttacactccttctctgcttccaccagagctgccatccgcgcagcttcattctttgctagcctggattcctcctgcagaagctggatcttattctccaagagctcataaacatgctccgtctcctgctgtcgctcctcaaactggcgtcggagctcagcttcattctgactgttgagattctccacatcagcccatgttttatccagatgctgtttcttgtcctggagttctcgtttcaagctctccacttcaaccttcagctcaatgttccgcttgtagatgtcctcccggctggcctcatacttctgttgcatgcgctcctccaggaagtagatgcgcagcttgaggctgaagttctccttcttcaggtcattgaggtgcttctcaaagtctcgaagagcctgggtctgtacctgagggggtttctcaaatgctctcaaggaatatgtctgcacaaacgggaccttttcaccacttctccagatctgtgactgcactggagggcctcgatctttagtgtcactaagaaaagctgctgtgtgactcgttctgggtaccatctccccatcatcctctgcaaaataatctctcatccagggtgtggccgccgcagctgcttcttcctcctcggccgctgctgcccagctcccggctggctccgggcgccgtctttcccggctcggggtctgccgtggggactgaggggttcgcgtcgcgtccccggaccggtaaggcgtgtagtgagcccggcgggacgcgcgacagcagcagccaaagtcgcatcggcggcggcagcaggacccgctgtctgtgcccttcatggatttcctgggcctggccaccccagtcctagctacggttcctgcttgttttcctggtgttttccgggactgccagggcgcatcctctgggcctggctgagcatccccgtcagttccctgggcctcctccgcggctgcctctgccacctgctccgcccagattgctttggtccttctcccgcagacacactcagctgcccttcatcctctgtcgtctccccattctctctccacccactgcctcattcccagatcccacgccgtttcttcctttctatccgctccaatgtcaccttctctttatttc

SEQ ID NO: 8822 - RNA, 7537 nt, Homo sapiens
  source 1..7537: mol_type = other RNA
aagtgtgcagggcactggtgctgctccgaagctcatgaatacctttgctgcctagcacctctgtgccttgggcttcaaggccagggaagctgcacgctgatctcacaagagacactatctttttgaccagcagcttgccctccgcaatctgctgtcttagggcactgtagtcatcaatgtggccaatgacatggcggccatgcttattggcaaaggagccatcagtagcatcaccctctagcttgggaggggtcttcattactggagaagtatccaaacccaagccatttgctctgttgattatgggcgtttctgagccaggagtagaggaagcagagctggggaagaccagagctggggaattcataccaacatcccggactggaggggacacagctgaatcttggaggagcagctgcttgtttccagggtcagtgctggctgggaagttctggttaatggaggaggggctgaggctggctttgccagcaccgctctccagctgctgttgcagctgcagtcgcagacaattgttcccctgaatgctctgctccagctgccctctcagagctcgtacctctgccaccaggtggctcaggtcactgctcaaagggatttggtgacaggcatccaggctgtaagctttcagccccttcttggaattgccataaagtgcctcgtagatttgtagctctgactggagggactcaaagagctgctgtttctcttcacactgttgctgcaggagaaccagcttgtgctgcagtctggagtcgttttcctggagggaaagacgttcctccctgaaatgcaagacctcttgctgcttctccctcaagtcttccaaaagctgctgcctttccaccttctggtgctccagctccttttccagctcttgaaggtgggatcgagaggacagcagagcctccctcaggctttctgtttcctgggagtgctctctggaaacatgactcagttgagcctgaagtcttcgattgtcttccctgaggactctgttctcattgcagagctgaggtatggactccaggccctgactgtagaagttagaagtggatccccttccacgagcagtagaggtcagccggtgttccagttgctcccgtaggcggtcattgatgcagatggattcctccaggcgctggcgcaggttccggatttcaccaagatgctcttccagcaggtcagcccctgtgggtttggagttaagctggtacacagaggagcctgaggataggtccccagatacactccctttctgaggcctcatcacatcccacttgccactgctgcccaggtacccaggctctaggattcttcccagttctatggtgccccttggaggagagtgaggctgggcagagttgaggtagtaggaagagtcggcttccaagtcgttgctcagcaatgtagctgtggaagcaggaggaacagtgctggcactttctcccaactgcttctgcagcatctgtagctcctgctgagcctcagccaaggagaccactggtgtctcacagcagccaaggaggagagggccagtggggctgaaaggcaggaagctggatggagctgagggcaatggtgcctgaggaaggctagccagcttgggtatggagtgaaaatgaaagcctgaatgggcctggttggcctccttgggggtattctggggagttggcaagctgatggggttgctgttggattcggccttagccccctgagatgcactggttgatgatggtttagaagacaacacagcagaatgactcgaatgatggatggaatctgagtgactgggagaagctttcttctcttcatagtgtgtgtactcgctgactatgtccatgtcagagcaggcttccagttcatcagacaggaaagaggtgctgctgggagagcggtgggagtcagacaaggcatggctgctggagggtgtgagggaccgagcatccagcttggcctgcaggacttcaatcactttctccttctcctgcagctccctgctgagcctgagggccagtggctcaagtccagcttgatctttctcacttttatgatccttggtgctgagtttgctggtgagcctctctgtcagctggcttccctgggcgagttgctcccggaagctctgtcccaggtagtagtcaatgtcattgctccttaggagatcctcaaaagattttactgtatcttttgcatgccgggtgataagataacaaatacctctcccttctcgtattttttgccgtaggtaagacagttcccgggcctgatcctgaatcagggaatcatatttcccaggccacgaggctgatctcagctcctcagccagcttctcttctagtccattttttgggagctgggcctccagctgggatactctctggatgagactctccaggtcctttttggcctgaagccctggagagtagaaagccccagtgccatcagacagccacccctcatcctcatcagggacactatgaggtgaagacccctccaaggtgccaacagctctcagcttccggggtctttccagactagacgaataatcacttgtaactgagagggaccggacccggctcttgaggttttgaatgaccttgttggcattctgcagctgggccttcagatctttgatgtcctttcgtaggaccaagatgttttctgactttccatatacccggaactcttcctgcttccctagctggttctccaagggcttcctctcagaggaactagccagtgttgagccccggcgtccctgctcagagcacagcccctccatcaggaccatttccttgaggctgttgtgctcctcacactcaggactggtggtttcctcccgttcagcctcattctcgcttcggccacaagtctcatagcccaggtcctggaggtccacctggatctgcttgctgtcctgcttcaccaaggattcactaagcataactctgtatttctccagctcgttagcctgagcaaagacagtggcttctgatagcagcagcttctcctggagatcttgatagcgttgtttgcattgtgacagctgggagcgcaggtgctgggtggaccctggtaggctaaacgctgactgaggcccagggtcacgaggctgggactggttatccaattggtgggcatccactgtgaaggtagccccaaggtcaaggctctggggtctggggaaaggcctcacagtcacattcccctcctcttggtgttggtgcttcccaggggaaccaaccagttctgtgtttattctttcaatggtgctggtcagatgcacaaggagctctggagtaagtttactattcccttccttgctactcagcacaagttgttctttgaggaggttgatgatattgtgggcattcttcagttttccctggagctttctgaactcagcctgaaggctactctcactcagaccctctttggttaccacagtctcaaccatcacctcgcccttctccttgtcttcctcgatctcccatccatcagacattgcttctcccatctgctctttcagctccgcattctcaaggcaaaggctcagcatggtgttcctgatgtgggacactgaggagaatcctgcttcctcaatttgagcctttagctccttcagttcctcctcagctttcctcttctcttctaagtgctggtggaactcagccctcaggtggagcatttcttcctgaagacacctgttactgtcccctcccatcggagaaggaggggaaaaagatgggttctgggtctccacagttgccagacttttctccaaagccaccttgacaagttgctggtgactatggtgtgcagcctcctcctcaatactgtcagtgaactcagtgcttgtatcttcggtgtcatcccctgcagctgcacctccaatggcggccagggtctccagcctgtttaagcgctccaagcttcttccaagaacttcttctagccgactgcgtaacacctgagccccttccagttccacctgcagagttcggtctctctcagagctctctggatgggcatggaacttcaccagactgctatagagctgtctctctgcttgtaaggcctcattgagccgactccgttcatctactagtccttctagcatcagcagcaactgttgtcttcggtttcctgaaatttcttgaccctgggattctactgaagcaactttttcccgaagaagtaagacttcctgggtcaggcgttccatagctggtatgtcttcaggatcaaccagttgcatttgcaggtcctttatgagatcttctttaatctgtatgttcctggtcagagactccatatcagcagcctgcacctgcagctcttcttcctgcacagccatcatggactgtagagcagaaagttccatctgactttctctttcttttttagccatgagttcaagttcctctttggcattactcagttctttttccagccctgcaactgtgtccaagtctcctaatgtggatctgggtatgctgacatcctctttggcagtcaatgaagtgctatcatctctggaaggtatctgcattgaaccttgatcagtctgttttccaagacggccagtgggggtaacttcagcttgttggttagagatgggtgcttgggacatcagggagtctctccctcctaaatattggcgcagggcctgtaattctgaatttctttccattaaggcttgcaccaacttctctgcagcagcttggctttcctgctccctggtgctcacagactgaagcaggccttgaatctccatttcatgttccagcacttgtttatttcgatcacttagaaggtcctgcagcatcctttcctttcgctgtagacgctggcacagctcctctgctatctcactctgccctggtccaagtttgcagagcagtgttgcactaagatcctccacttctttgttcctatcatgaagagacgtctgtaactgctgaatgatactctcttgttccttctgccaacggctaaatttggtttccatttcttctttcagccactggaggttttgacaggtagtagataactgttccacttccaggcctttggccctcaggagactctccatactttgcatagtagcttcattggaggagaggacatcgcgcagtctctctaagtcatgatctcgctctctcacagcaagacgaagctggcgcagttctttttctttctcttctagagcagagaatttttcatctatagcccgctccagagcaacagctttatcatgtattcgctggcgaagtttctcaagcaacatttcatttgcttcaagggttttgtctgagttatctcgatactgtaggagctcccgaaattcctgaagcaactgctccttgtgactcagactatggtttaggtgctggatgttttgttcctgggttcgaatctcattgtatttttcagcctcccaggcacgaagctgttggctcttattctgcaattcttcttgtagctgctgcaaggcttttcgcaattcctggttatgtttccaagaagcctctttctgctgttcactctcgtgtgctgcagcctctacaaattgcacacattgtttggcatcagccagttggcgctctttctgtcgtaccaccctctggagcttctgtatttcaagttggctgcagaataaagcactctgaagatcaagcagagctacctgttgctgagctggagaagtaccctctgagctgtgaagttgtccaagctggctttggtgcagcatttctcgaagctttgccattgtgtcattttgaccttcaattacctggtacaactcctcagtctcacgttccctgcttttcagagtttccttgaggttctgaattgtaccatcttgcttttgagacgactcctgagcacactttagttcatagctcatttcattaagtttctcttgaagaatcttgttggtggcctctgtttgctggattttttcctggagttctgccaagtgggaatcagatacagactgctgagttatagtggtctcatgtgaattcagcttttgttgtttcagcaactcttcagtcatgggctggacccggagcggcaaataatcttcacagagatcatcccacagctcctgcaggtctgaaagctccaagggataactcacaggtgtcttgtaaaggggtttcaaagacctgttaaggaaaccggaactaactccatctgtcatgctagggccaggcttggctccaggtaggctggatttcactggaatcggaagcctgctccctcgggggctctggatgggcttataatcaagacctttaatcatgctaagagctaattccagcttgtgattacacccatgctgcggagcctgatcatctgaacaacagtcacactttccaagttcctttgcacttctctcagtctcctcatctttctgttgtggagggctagcctggacgcttgcatccaaagattccacagaggaaccaggcgtctcttcctccatgctttctccatctgggggtacctttgtgcttgctaagtcgggtggcccaacctcagacaacgctggttcttcagtgcaaatgctggtcgaccacctgctagaagggccgcaggagatacttctggccacctttcgaggtaccttacaaatggcttcatagtcagaatcagcaacccgcaaagcggcacaaccacggcatctcctgggtcggtttccagggccttctgaaccatggcagctgtgtggctcctggatctgatcctcattctccacccagcactcaaaccctgaataggcgaagtcctcctggagcagtgcagagtatctcgcatcgggtaagacggacatgtcaaccgtcccattccccgccttgatctccgcgccagagtcatcgttattcttccgatacatactggcaatgcagaacttgaggcgatccttctccagtagcagcttttgcaagcgctcaatagaaagcgcttcaatccgggcaataactgtgtcgaatcgatagattcgatcaagcatgaaagcacacttgctgcaagcgaactcggctttgccatcgcgggggacatccttgcccaagacgtgcgaaagcagaacctggagattgagcttggacgccgtgtggaagatccagcgccgctggtttccacacagctctcgggcacagatcctgcaaatctccttcatcttccctcctagcgggtggcaagcttcccgaggcggcggcggcggcggctactgggtgaccactcaatggctcttcgccgcgctctgtctcccgcctcggtggtctccggtcagcatggcacagcccagtggggtccccactctgcaggggcgcgcccctgccccgcgcgccgactccgggtaccagagccgtcagccccgcccctcgggcagggggcgggcgtggaaacgcctaagaggatgctgagtgacagaggcgcaggccgcgctccgaccctgccatgtctctccccagctgtctctcccgccagccgccgcgtcctc

SEQ ID NO: 8823 - RNA, 7620 nt, Homo sapiens
  source 1..7620: mol_type = other RNA
aagtgtgcagggcactggtgctgctccgaagctcatgaatacctttgctgcctagcacctctgtgccttgggcttcaaggccagggaagctgcacgctgatctcacaagagacactatctttttgaccagcagcttgccctccgcaatctgctgtcttagggcactgtagtcatcaatgtggccaatgacatggcggccatgcttattggcaaaggagccatcagtagcatcaccctctagcttgggaggggtcttcattactggagaagtatccaaacccaagccatttgctctgttgattatgggcgtttctgagccaggagtagaggaagcagagctggggaagaccagagctggggaattcataccaacatcccggactggaggggacacagctgaatcttggaggagcagctgcttgtttccagggtcagtgctggctgggaagttctggttaatggaggaggggctgaggctggctttgccagcaccgctctccagctgctgttgcagctgcagtcgcagacaattgttcccctgaatgctctgctccagctgccctctcagagctcgtacctctgccaccaggtggctcaggtcactgctcaaagggatttggtgacaggcatccaggctgtaagctttcagccccttcttggaattgccataaagtgcctcgtagatttgtagctctgactggagggactcaaagagctgctgtttctcttcacactgttgctgcaggagaaccagcttgtgctgcagtctggagtcgttttcctggagggaaagacgttcctccctgaaatgcaagacctcttgctgcttctccctcaagtcttccaaaagctgctgcctttccaccttctggtgctccagctccttttccagctcttgaaggtgggatcgagaggacagcagagcctccctcaggctttctgtttcctgggagtgctctctggaaacatgactcagttgagcctgaagtcttcgattgtcttccctgaggactctgttctcattgcagagctgaggtatggactccaggccctgactgtagaagttagaagtggatccccttccacgagcagtagaggtcagccggtgttccagttgctcccgtaggcggtcattgatgcagatggattcctccaggcgctggcgcaggttccggatttcaccaagatgctcttccagcaggtcagcccctgtgggtttggagttaagctggtacacagaggagcctgaggataggtccccagatacactccctttctgaggcctcatcacatcccacttgccactgctgcccaggtacccaggctctaggattcttcccagttctatggtgccccttggaggagagtgaggctgggcagagttgaggtagtaggaagagtcggcttccaagtcgttgctcagcaatgtagctgtggaagcaggaggaacagtgctggcactttctcccaactgcttctgcagcatctgtagctcctgctgagcctcagccaaggagaccactggtgtctcacagcagccaaggaggagagggccagtggggctgaaaggcaggaagctggatggagctgagggcaatggtgcctgaggaaggctagccagcttgggtatggagtgaaaatgaaagcctgaatgggcctggttggcctccttgggggtattctggggagttggcaagctgatggggttgctgttggattcggccttagccccctgagatgcactggttgatgatggtttagaagacaacacagcagaatgactcgaatgatggatggaatctgagtgactgggagaagctttcttctcttcatagtgtgtgtactcgctgactatgtccatgtcagagcaggcttccagttcatcagacaggaaagaggtgctgctgggagagcggtgggagtcagacaaggcatggctgctggagggtgtgagggaccgagcatccagcttggcctgcaggacttcaatcactttctccttctcctgcagctccctgctgagcctgagggccagtggctcaagtccagcttgatctttctcacttttatgatccttggtgctgagtttgctggtgagcctctctgtcagctggcttccctgggcgagttgctcccggaagctctgtcccaggtagtagtcaatgtcattgctccttaggagatcctcaaaagattttactgtatcttttgcatgccgggtgataagataacaaatacctctcccttctcgtattttttgccgtaggtaagacagttcccgggcctgatcctgaatcagggaatcatatttcccaggccacgaggctgatctcagctcctcagccagcttctcttctagtccattttttgggagctgggcctccagctgggatactctctggatgagactctccaggtcctttttggcctgaagccctggagagtagaaagccccagtgccatcagacagccacccctcatcctcatcagggacactatgaggtgaagacccctccaaggtgccaacagctctcagcttccggggtctttccagactagacgaataatcacttgtaactgagagggaccggacccggctcttgaggttttgaatgaccttgttggcattctgcagctgggccttcagatctttgatgtcctttcgtaggaccaagatgttttctgactttccatatacccggaactcttcctgcttccctagctggttctccaagggcttcctctcagaggaactagccagtgttgagccccggcgtccctgctcagagcacagcccctccatcaggaccatttccttgaggctgttgtgctcctcacactcaggactggtggtttcctcccgttcagcctcattctcgcttcggccacaagtctcatagcccaggtcctggaggtccacctggatctgcttgctgtcctgcttcaccaaggattcactaagcataactctgtatttctccagctcgttagcctgagcaaagacagtggcttctgatagcagcagcttctcctggagatcttgatagcgttgtttgcattgtgacagctgggagcgcaggtgctgggtggaccctggtaggctaaacgctgactgaggcccagggtcacgaggctgggactggttatccaattggtgggcatccactgtgaaggtagccccaaggtcaaggctctggggtctggggaaaggcctcacagtcacattcccctcctcttggtgttggtgcttcccaggggaaccaaccagttctgtgtttattctttcaatggtgctggtcagatgcacaaggagctctggagtaagtttactattcccttccttgctactcagcacaagttgttctttgaggaggttgatgatattgtgggcattcttcagttttccctggagctttctgaactcagcctgaaggctactctcactcagaccctctttggttaccacagtctcaaccatcacctcgcccttctccttgtcttcctcgatctcccatccatcagacattgcttctcccatctgctctttcagctccgcattctcaaggcaaaggctcagcatggtgttcctgatgtgggacactgaggagaatcctgcttcctcaatttgagcctttagctccttcagttcctcctcagctttcctcttctcttctaagtgctggtggaactcagccctcaggtggagcatttcttcctgaagacacctgttactgtcccctcccatcggagaaggaggggaaaaagatgggttctgggtctccacagttgccagacttttctccaaagccaccttgacaagttgctggtgactatggtgtgcagcctcctcctcaatactgtcagtgaactcagtgcttgtatcttcggtgtcatcccctgcagctgcacctccaatggcggccagggtctccagcctgtttaagcgctccaagcttcttccaagaacttcttctagccgactgcgtaacacctgagccccttccagttccacctgcagagttcggtctctctcagagctctctggatgggcatggaacttcaccagactgctatagagctgtctctctgcttgtaaggcctcattgagccgactccgttcatctactagtccttctagcatcagcagcaactgttgtcttcggtttcctgaaatttcttgaccctgggattctactgaagcaactttttcccgaagaagtaagacttcctgggtcaggcgttccatagctggtatgtcttcaggatcaaccagttgcatttgcaggtcctttatgagatcttctttaatctgtatgttcctggtcagagactccatatcagcagcctgcacctgcagctcttcttcctgcacagccatcatggactgtagagcagaaagttccatctgactttctctttcttttttagccatgagttcaagttcctctttggcattactcagttctttttccagccctgcaactgtgtccaagtctcctaatgtggatctgggtatgctgacatcctctttggcagtcaatgaagtgctatcatctctggaaggtatctgcattgaaccttgatcagtctgttttccaagacggccagtgggggtaacttcagcttgttggttagagatgggtgcttgggacatcagggagtctctccctcctaaatattggcgcagggcctgtaattctgaatttctttccattaaggcttgcaccaacttctctgcagcagcttggctttcctgctccctggtgctcacagactgaagcaggccttgaatctccatttcatgttccagcacttgtttatttcgatcacttagaaggtcctgcagcatcctttcctttcgctgtagacgctggcacagctcctctgctatctcactctgccctggtccaagtttgcagagcagtgttgcactaagatcctccacttctttgttcctatcatgaagagacgtctgtaactgctgaatgatactctcttgttccttctgccaacggctaaatttggtttccatttcttctttcagccactggaggttttgacaggtagtagataactgttccacttccaggcctttggccctcaggagactctccatactttgcatagtagcttcattggaggagaggacatcgcgcagtctctctaagtcatgatctcgctctctcacagcaagacgaagctggcgcagttctttttctttctcttctagagcagagaatttttcatctatagcccgctccagagcaacagctttatcatgtattcgctggcgaagtttctcaagcaacatttcatttgcttcaagggttttgtctgagttatctcgatactgtaggagctcccgaaattcctgaagcaactgctccttgtgactcagactatggtttaggtgctggatgttttgttcctgggttcgaatctcattgtatttttcagcctcccaggcacgaagctgttggctcttattctgcaattcttcttgtagctgctgcaaggcttttcgcaattcctggttatgtttccaagaagcctctttctgctgttcactctcgtgtgctgcagcctctacaaattgcacacattgtttggcatcagccagttggcgctctttctgtcgtaccaccctctggagcttctgtatttcaagttggctgcagaataaagcactctgaagatcaagcagagctacctgttgctgagctggagaagtaccctctgagctgtgaagttgtccaagctggctttggtgcagcatttctcgaagctttgccattgtgtcattttgaccttcaattacctggtacaactcctcagtctcacgttccctgcttttcagagtttccttgaggttctgaattgtaccatcttgcttttgagacgactcctgagcacactttagttcatagctcatttcattaagtttctcttgaagaatcttgttggtggcctctgtttgctggattttttcctggagttctgccaagtgggaatcagatacagactgctgagttatagtggtctcatgtgaattcagcttttgttgtttcagcaactcttcagtcatgggctggacccggagcggcaaataatcttcacagagatcatcccacagctcctgcaggtctgaaagctccaagggataactcacaggtgtcttgtaaaggggtttcaaagacctgttaaggaaaccggaactaactccatctgtcatgctagggccaggcttggctccaggtaggctggatttcactggaatcggaagcctgctccctcgggggctctggatgggcttataatcaagacctttaatcatgctaagagctaattccagcttgtgattacacccatgctgcggagcctgatcatctgaacaacagtcacactttccaagttcctttgcacttctctcagtctcctcatctttctgttgtggagggctagcctggacgcttgcatccaaagattccacagaggaaccaggcgtctcttcctccatgctttctccatctgggggtacctttgtgcttgctaagtcgggtggcccaacctcagacaacgctggttcttcagtgcaaatgctggtcgaccacctgctagaagggccgcaggagatacttctggccacctttcgaggtaccttacaaatggcttcatagtcagaatcagcaacccgcaaagcggcacaaccacggcatctcctgggtcggtttccagggccttctgaaccatggcagctgtgtggctcctggatctgatcctcattctccacccagcactcaaaccctgaataggcgaagtcctcctggagcagtgcagagtatctcgcatcgggtaagacggacatgtcaaccgtcccattccccgccttgatctccgcgccagagtcatcgttattcttccgatacatactggcaatgcagaacttgaggcgatccttctccagtagcagcttttgcaagcgctcaatagaaagcgcttcaatccgggcaataactgtgtcgaatcgatagattcgatcaagcatgaaagcacacttgctgcaagcgaactcggctttgccatcgcgggggacatccttgcccaagacgtgcgaaagcagaacctggagattgagcttggacgccgtgtggaagatccagcgccgctggtttccacacagctctcgggcacagatcctgcaaatctccttcatcttccctcctagcgggtggcaagcttcccgaggcggcggcggcggcggctactgggtgaccactcaatggctcttcgccgcgctctgtctcccgcctcggtggtctccggtcagcatggcacagcccagtggggtccccactctgcaggggcgcgcccctgccccgcgcgccgactccgggtaccagagccgtcagccccgcccctcgggcagggggcgggcgtggaaacgcctaagaggatgctgagtgacagaggcgcaggccgcgctccgaccctgccatgtctctccccagctgtctctcccgccagccgccgcgtcctcaacgtcctccccttttagcagactgggctcccggagcagcagcggccggccgcgcagacgcaaagcctcggggatggaggatc

SEQ ID NO: 8824 - RNA, 6517 nt, Homo sapiens
  source 1..6517: mol_type = other RNA
aagtgtgcagggcactggtgctgctccgaagctcatgaatacctttgctgcctagcacctctgtgccttgggcttcaaggccagggaagctgcacgctgatctcacaagagacactatctttttgaccagcagcttgccctccgcaatctgctgtcttagggcactgtagtcatcaatgtggccaatgacatggcggccatgcttattggcaaaggagccatcagtagcatcaccctctagcttgggaggggtcttcattactggagaagtatccaaacccaagccatttgctctgttgattatgggcgtttctgagccaggagtagaggaagcagagctggggaagaccagagctggggaattcataccaacatcccggactggaggggacacagctgaatctttcagccccttcttggaattgccataaagtgcctcgtagatttgtagctctgactggagggactcaaagagctgctgtttctcttcacactgttgctgcaggagaaccagcttgtgctgcagtctggagtcgttttcctggagggaaagacgttcctccctgaaatgcaagacctcttgctgcttctccctcaagtcttccaaaagctgctgcctttccaccttctggtgctccagctccttttccagctcttgaaggtgggatcgagaggacagcagagcctccctcaggctttctgtttcctgggagtgctctctggaaacatgactcagttgagcctgaagtcttcgattgtcttccctgaggactctgttctcattgcagagctgaggtatggactccaggccctgactgtagaagttagaagtggatccccttccacgagcagtagaggtcagccggtgttccagttgctcccgtaggcggtcattgatgcagatggattcctccaggcgctggcgcaggttccggatttcaccaagatgctcttccagcaggtcagcccctgtgggtttggagttaagctggtacacagaggagcctgaggataggtccccagatacactccctttctgaggcctcatcacatcccacttgccactgctgcccaggtacccaggctctaggattcttcccagttctatggtgccccttggaggagagtgaggctgggcagagttgaggtagtaggaagagtcggcttccaagtcgttgctcagcaatgtagctgtggaagcaggaggaacagtgctggcacctgaatgggcctggttggcctccttgggggtattctggggagttggcaagctgatggggttgctgttggattcggccttagccccctgagatgcactggttgatgatggtttagaagacaacacagcagaatgactcgaatgatggatggaatctgagtgactgggagaagctttcttctcttcatagtgtgtgtactcgctgactatgtccatgtcagagcaggcttccagttcatcagacaggaaagaggtgctgctgggagagcggtgggagtcagacaaggcatggctgctggagggtgtgagggaccgagcatccagcttggcctgcaggacttcaatcactttctccttctcctgcagctccctgctgagcctgagggccagtggctcaagtccagcttgatctttctcacttttatgatccttggtgctgagtttgctggtgagcctctctgtcagctggcttccctgggcgagttgctcccggaagctctgtcccaggtagtagtcaatgtcattgctccttaggagatcctcaaaagattttactgtatcttttgcatgccgggtgataagataacaaatacctctcccttctcgtattttttgccgtaggtaagacagttcccgggcctgatcctgaatcagggaatcatatttcccaggccacgaggctgatctcagctcctcagccagcttctcttctagtccattttttgggagctgggcctccagctgggatactctctggatgagactctccaggtcctttttggcctgaagccctggagagtagaaagccccagtgccatcagacagccacccctcatcctcatcagggacactatgaggtgaagacccctccaaggtgccaacagctctcagcttccggggtctttccagactagacgaataatcacttgtaactgagagggaccggacccggctcttgaggttttgaatgaccttgttggcattctgcagctgggccttcagatctttgatgtcctttcgtaggaccaagatgttttctgactttccatatacccggaactcttcctgcttccctagctggttctccaagggcttcctctcagaggaactagccagtgttgagccccggcgtccctgctcagagcacagcccctccatcaggaccatttccttgaggctgttgtgctcctcacactcaggactggtggtttcctcccgttcagcctcattctcgcttcggccacaagtctcatagcccaggtcctggaggtccacctggatctgcttgctgtcctgcttcaccaaggattcacctgtaagcataactctgtatttctccagctcgttagcctgagcaaagacagtggcttctgatagcagcagcttctcctggagatcttgatagcgttgtttgcattgtgacagctgggagcgcaggtgctgggtggaccctggtaggctaaacgctgactgaggcccagggtcacgaggctgggactggttatccaactcgcccttctccttgtcttcctcgatctcccatccatcagacattgcttctcccatctgctctttcagctccgcattctcaaggcaaaggctcagcatggtgttcctgatgtgggacactgaggagaatcctgcttcctcaatttgagcctttagctccttcagttcctcctcagctttcctcttctcttctaagtgctggtggaactcagccctcaggtggagcatttcttcctgaagacacctgttactgtcccctcccatcggagaaggaggggaaaaagatgggttctgggtctccacagttgccagacttttctccaaagccaccttgacaagttgctggtgactatggtgtgcagcctcctcctcaatactgtcagtgaactcagtgcttgtatcttcggtgtcatcccctgcagctgcacctccaatggcggccagggtctccagcctgtttaagcgctccaagcttcttccaagaacttcttctagccgactgcgtaacacctgagccccttccagttccacctgcagagttcggtctctctcagagctctctggatgggcatggaacttcaccagactgctatagagctgtctctctgcttgtaaggcctcattgagccgactccgttcatctactagtccttctagcatcagcagcaactgttgtcttcggtttcctgaaatttcttgaccctgggattctactgaagcaactttttcccgaagaagtaagacttcctgggtcaggcgttccatagctggtatgtcttcaggatcaaccagttgcatttgcaggtcctttatgagatcttctttaatctgtatgttcctggtcagagactccatatcagcagcctgcacctgcagctcttcttcctgcacagccatcatggactgtagagcagaaagttccatctgactttctctttcttttttagccatgagttcaagttcctctttggcattactcagttctttttccagccctgcaactgtgtccaagtctcctaatgtggatctgggtatgctgacatcctctttggcagtcaatgaagtgctatcatctctggaaggtatctgcattgaaccttgatcagtctgttttccaagacggccagtgggggtaacttcagcttgttggttagagatgggtgcttgggacatcagggagtctctccctcctaaatattggcgcagggcctgtaattctgaatttctttccattaaggcttgcaccaacttctctgcagcagcttggctttcctgctccctggtgctcacagactgaagcaggccttgaatctccatttcatgttccagcacttgtttatttcgatcacttagaaggtcctgcagcatcctttcctttcgctgtagacgctggcacagctcctctgctatctcactctgccctggtccaagtttgcagagcagtgttgcactaagatcctccacttctttgttcctatcatgaagagacgtctgtaactgctgaatgatactctcttgttccttctgccaacggctaaatttggtttccatttcttctttcagccactggaggttttgacaggtagtagataactgttccacttccaggcctttggccctcaggagactctccatactttgcatagtagcttcattggaggagaggacatcgcgcagtctctctaagtcatgatctcgctctctcacagcaagacgaagctggcgcagttctttttctttctcttctagagcagagaatttttcatctatagcccgctccagagcaacagctttatcatgtattcgctggcgaagtttctcaagcaacatttcatttgcttcaagggttttgtctgagttatctcgatactgtaggagctcccgaaattcctgaagcaactgctccttgtgactcagactatggtttaggtgctggatgttttgttcctgggttcgaatctcattgtatttttcagcctcccaggcacgaagctgttggctcttattctgcaattcttcttgtagctgctgcaaggcttttcgcaattcctggttatgtttccaagaagcctctttctgctgttcactctcgtgtgctgcagcctctacaaattgcacacattgtttggcatcagccagttggcgctctttctgtcgtaccaccctctggagcttctgtatttcaagttggctgcagaataaagcactctgaagatcaagcagagctacctgttgctgagctggagaagtaccctctgagctgtgaagttgtccaagctggctttggtgcagcatttctcgaagctttgccattgtgtcattttgaccttcaattacctggtacaactcctcagtctcacgttccctgcttttcagagtttccttgaggttctgaattgtaccatcttgcttttgagacgactcctgagcacactttagttcatagctcatttcattaagtttctcttgaagaatcttgttggtggcctctgtttgctggattttttcctggagttctgccaagtgggaatcagatacagactgctgagttatagtggtctcatgtgaattcagcttttgttgtttcagcaactcttcagtcatgggctgcacttccatgctagttggctcctccaacagatgtagcagttgttgtttctcccgagatagctgttctacaagcctctcctgggcagccaggctctgattcagttcttcaattctcttgtccctctgggccagggcctcagtgtattggtcgggcttgacctggtctcctggtacatcttcccagtttttggtgactcccttcagtttctctgagagctccaggttacactccttctctgcttccaccagagctgccatccgcgcagcttcattctttgctagcctggattcctcctgcagaagctggatcttattctccaagagctcataaacatgctccgtctcctgctgtcgctcctcaaactggcgtcggagctcagcttcattctgactgttgagattctccacatcagcccatgttttatccagatgctgtttcttgtcctggagttctcgtttcaagctctccacttcaaccttcagctcaatgttccgcttgtagatgtcctcccggctggcctcatacttctgttgcatgcgctcctccaggaagtagatgcgcagcttgaggctgaagttctccttcttcaggtcattgaggtgcttctcaaagtctcgaagagcctgggtctgtacctgagggggtttctcaaatgctctcaaggaatatgtctgcacaaacgggaccttttcaccacttctccagatctgtgactgcactggagggcctcgatctttagtgtcactaagaaaagctgctgtgtgactcgttctgggtaccatctccccatcatcctctgcaaaataatctctcgtccaggtctgctccattttccaggctctttccttagtctcaggacgctcctcacccgggaggggaagcagcctgggaaaatgagaagccttgcccacgaatctccagcgcaaaaggcagcagctttttcctccccagctcctttctgcgtcggcggcgaagagagagctctgctccctgcttttttagaaaatggatttgacgtggccgaacctgcggctagccgtgcgacccgcacaagggagggactgttctcagtaggaggctggactcagagcggcgcggcgcccggggctgtttcgtgagctggagccagcggctgcccgggccgcggtgcgcgcactctccaggctgagacacgactg

SEQ ID NO: 8825 - RNA, 6867 nt, Homo sapiens
  source 1..6867: mol_type = other RNA
aagtgtgcagggcactggtgctgctccgaagctcatgaatacctttgctgcctagcacctctgtgccttgggcttcaaggccagggaagctgcacgctgatctcacaagagacactatctttttgaccagcagcttgccctccgcaatctgctgtcttagggcactgtagtcatcaatgtggccaatgacatggcggccatgcttattggcaaaggagccatcagtagcatcaccctctagcttgggaggggtcttcattactggagaagtatccaaacccaagccatttgctctgttgattatgggcgtttctgagccaggagtagaggaagcagagctggggaagaccagagctggggaattcataccaacatcccggactggaggggacacagctgaatctttcagccccttcttggaattgccataaagtgcctcgtagatttgtagctctgactggagggactcaaagagctgctgtttctcttcacactgttgctgcaggagaaccagcttgtgctgcagtctggagtcgttttcctggagggaaagacgttcctccctgaaatgcaagacctcttgctgcttctccctcaagtcttccaaaagctgctgcctttccaccttctggtgctccagctccttttccagctcttgaaggtgggatcgagaggacagcagagcctccctcaggctttctgtttcctgggagtgctctctggaaacatgactcagttgagcctgaagtcttcgattgtcttccctgaggactctgttctcattgcagagctgaggtatggactccaggccctgactgtagaagttagaagtggatccccttccacgagcagtagaggtcagccggtgttccagttgctcccgtaggcggtcattgatgcagatggattcctccaggcgctggcgcaggttccggatttcaccaagatgctcttccagcaggtcagcccctgtgggtttggagttaagctggtacacagaggagcctgaggataggtccccagatacactccctttctgaggcctcatcacatcccacttgccactgctgcccaggtacccaggctctaggattcttcccagttctatggtgccccttggaggagagtgaggctgggcagagttgaggtagtaggaagagtcggcttccaagtcgttgctcagcaatgtagctgtggaagcaggaggaacagtgctggcacctgaatgggcctggttggcctccttgggggtattctggggagttggcaagctgatggggttgctgttggattcggccttagccccctgagatgcactggttgatgatggtttagaagacaacacagcagaatgactcgaatgatggatggaatctgagtgactgggagaagctttcttctcttcatagtgtgtgtactcgctgactatgtccatgtcagagcaggcttccagttcatcagacaggaaagaggtgctgctgggagagcggtgggagtcagacaaggcatggctgctggagggtgtgagggaccgagcatccagcttggcctgcaggacttcaatcactttctccttctcctgcagctccctgctgagcctgagggccagtggctcaagtccagcttgatctttctcacttttatgatccttggtgctgagtttgctggtgagcctctctgtcagctggcttccctgggcgagttgctcccggaagctctgtcccaggtagtagtcaatgtcattgctccttaggagatcctcaaaagattttactgtatcttttgcatgccgggtgataagataacaaatacctctcccttctcgtattttttgccgtaggtaagacagttcccgggcctgatcctgaatcagggaatcatatttcccaggccacgaggctgatctcagctcctcagccagcttctcttctagtccattttttgggagctgggcctccagctgggatactctctggatgagactctccaggtcctttttggcctgaagccctggagagtagaaagccccagtgccatcagacagccacccctcatcctcatcagggacactatgaggtgaagacccctccaaggtgccaacagctctcagcttccggggtctttccagactagacgaataatcacttgtaactgagagggaccggacccggctcttgaggttttgaatgaccttgttggcattctgcagctgggccttcagatctttgatgtcctttcgtaggaccaagatgttttctgactttccatatacccggaactcttcctgcttccctagctggttctccaagggcttcctctcagaggaactagccagtgttgagccccggcgtccctgctcagagcacagcccctccatcaggaccatttccttgaggctgttgtgctcctcacactcaggactggtggtttcctcccgttcagcctcattctcgcttcggccacaagtctcatagcccaggtcctggaggtccacctggatctgcttgctgtcctgcttcaccaaggattcacctgtaagcataactctgtatttctccagctcgttagcctgagcaaagacagtggcttctgatagcagcagcttctcctggagatcttgatagcgttgtttgcattgtgacagctgggagcgcaggtgctgggtggaccctggtaggctaaacgctgactgaggcccagggtcacgaggctgggactggttatccaactcgcccttctccttgtcttcctcgatctcccatccatcagacattgcttctcccatctgctctttcagctccgcattctcaaggcaaaggctcagcatggtgttcctgatgtgggacactgaggagaatcctgcttcctcaatttgagcctttagctccttcagttcctcctcagctttcctcttctcttctaagtgctggtggaactcagccctcaggtggagcatttcttcctgaagacacctgttactgtcccctcccatcggagaaggaggggaaaaagatgggttctgggtctccacagttgccagacttttctccaaagccaccttgacaagttgctggtgactatggtgtgcagcctcctcctcaatactgtcagtgaactcagtgcttgtatcttcggtgtcatcccctgcagctgcacctccaatggcggccagggtctccagcctgtttaagcgctccaagcttcttccaagaacttcttctagccgactgcgtaacacctgagccccttccagttccacctgcagagttcggtctctctcagagctctctggatgggcatggaacttcaccagactgctatagagctgtctctctgcttgtaaggcctcattgagccgactccgttcatctactagtccttctagcatcagcagcaactgttgtcttcggtttcctgaaatttcttgaccctgggattctactgaagcaactttttcccgaagaagtaagacttcctgggtcaggcgttccatagctggtatgtcttcaggatcaaccagttgcatttgcaggtcctttatgagatcttctttaatctgtatgttcctggtcagagactccatatcagcagcctgcacctgcagctcttcttcctgcacagccatcatggactgtagagcagaaagttccatctgactttctctttcttttttagccatgagttcaagttcctctttggcattactcagttctttttccagccctgcaactgtgtccaagtctcctaatgtggatctgggtatgctgacatcctctttggcagtcaatgaagtgctatcatctctggaaggtatctgcattgaaccttgatcagtctgttttccaagacggccagtgggggtaacttcagcttgttggttagagatgggtgcttgggacatcagggagtctctccctcctaaatattggcgcagggcctgtaattctgaatttctttccattaaggcttgcaccaacttctctgcagcagcttggctttcctgctccctggtgctcacagactgaagcaggccttgaatctccatttcatgttccagcacttgtttatttcgatcacttagaaggtcctgcagcatcctttcctttcgctgtagacgctggcacagctcctctgctatctcactctgccctggtccaagtttgcagagcagtgttgcactaagatcctccacttctttgttcctatcatgaagagacgtctgtaactgctgaatgatactctcttgttccttctgccaacggctaaatttggtttccatttcttctttcagccactggaggttttgacaggtagtagataactgttccacttccaggcctttggccctcaggagactctccatactttgcatagtagcttcattggaggagaggacatcgcgcagtctctctaagtcatgatctcgctctctcacagcaagacgaagctggcgcagttctttttctttctcttctagagcagagaatttttcatctatagcccgctccagagcaacagctttatcatgtattcgctggcgaagtttctcaagcaacatttcatttgcttcaagggttttgtctgagttatctcgatactgtaggagctcccgaaattcctgaagcaactgctccttgtgactcagactatggtttaggtgctggatgttttgttcctgggttcgaatctcattgtatttttcagcctcccaggcacgaagctgttggctcttattctgcaattcttcttgtagctgctgcaaggcttttcgcaattcctggttatgtttccaagaagcctctttctgctgttcactctcgtgtgctgcagcctctacaaattgcacacattgtttggcatcagccagttggcgctctttctgtcgtaccaccctctggagcttctgtatttcaagttggctgcagaataaagcactctgaagatcaagcagagctacctgttgctgagctggagaagtaccctctgagctgtgaagttgtccaagctggctttggtgcagcatttctcgaagctttgccattgtgtcattttgaccttcaattacctggtacaactcctcagtctcacgttccctgcttttcagagtttccttgaggttctgaattgtaccatcttgcttttgagacgactcctgagcacactttagttcatagctcatttcattaagtttctcttgaagaatcttgttggtggcctctgtttgctggattttttcctggagttctgccaagtgggaatcagatacagactgctgagttatagtggtctcatgtgaattcagcttttgttgtttcagcaactcttcagtcatgggctggacccggagcggcaaataatcttcacagagatcatcccacagctcctgcaggtctgaaagctccaagggataactcacaggtgtcttgtaaaggggtttcaaagacctgttaaggaaaccggaactaactccatctgtcatgctagggccaggcttggctccaggtaggctggatttcactggaatcggaagcctgctccctcgggggctctggatgggcttataatcaagacctttaatcatgctaagagctaattccagcttgtgattacacccatgctgcggagcctgatcatctgaacaacagtcacactttccaagttcctttgcacttctctcagtctcctcatctttctgttgtggagggctagcctggacgcttgcatccaaagattccacagaggaaccaggcgtctcttcctccatgctttctccatctgggggtacctttgtgcttgctaagtcgggtggcccaacctcagacaacgctggttcttcagtgcaaatgctggtcgaccacctgctagaagggccgcaggagatacttctggccacctttcgaggtaccttacaaatggcttcatagtcagaatcagcaacccgcaaagcggcacaaccacggcatctcctgggtcggtttccagggccttctgaaccatggcagctgtgtggctcctggatctgatcctcattctccacccagcactcaaaccctgaataggcgaagtcctcctggagcagtgcagagtatctcgcatcgggtaagacggacatgtcaaccgtcccattccccgccttgatctccgcgccagagtcatcgttattcttccgatacatactggcaatgcagaacttgaggcgatccttctccagtagcagcttttgcaagcgctcaatagaaagcgcttcaatccgggcaataactgtgtcgaatcgatagattcgatcaagcatgaaagcacacttgctgcaagcgaactcggctttgccatcgcgggggacatccttgcccaagacgtgcgaaagcagaacctggagattgagcttggacgccgtgtggaagatccagcgccgctggtttccacacagctctcgggcacagatcctgcaaatctccttcatcttccctcctagcgggtggcaagcttcccgaggcggcggcggcggcggctactgggtgaccactcaatggctcttcgccgcgctctgtctcccgcctcggtggtctccggtcagcatggcacagcccagtggggtccccactctgcaggggcgcgcccctgccccgcgcgccgactccgggtaccagagccgtcagccccgcccctcgggcagggggcgggcgtggaaacgcctaagaggatgctgagtgacagaggcgcaggccgcgctccgaccctgccatgtctctccccagctgtctctcccgccagccgccgcgtcctcaacgtcctccccttttagcagactgggctcccggagcagcagcggccggccgcgcagacgcaaagcctcggggatggaggatc

SEQ ID NO: 8826 - RNA, 7197 nt, Homo sapiens
  source 1..7197: mol_type = other RNA
aagtgtgcagggcactggtgctgctccgaagctcatgaatacctttgctgcctagcacctctgtgccttgggcttcaaggccagggaagctgcacgctgatctcacaagagacactatctttttgaccagcagcttgccctccgcaatctgctgtcttagggcactgtagtcatcaatgtggccaatgacatggcggccatgcttattggcaaaggagccatcagtagcatcaccctctagcttgggaggggtcttcattactggagaagtatccaaacccaagccatttgctctgttgattatgggcgtttctgagccaggagtagaggaagcagagctggggaagaccagagctggggaattcataccaacatcccggactggaggggacacagctgaatctttcagccccttcttggaattgccataaagtgcctcgtagatttgtagctctgactggagggactcaaagagctgctgtttctcttcacactgttgctgcaggagaaccagcttgtgctgcagtctggagtcgttttcctggagggaaagacgttcctccctgaaatgcaagacctcttgctgcttctccctcaagtcttccaaaagctgctgcctttccaccttctggtgctccagctccttttccagctcttgaaggtgggatcgagaggacagcagagcctccctcaggctttctgtttcctgggagtgctctctggaaacatgactcagttgagcctgaagtcttcgattgtcttccctgaggactctgttctcattgcagagctgaggtatggactccaggccctgactgtagaagttagaagtggatccccttccacgagcagtagaggtcagccggtgttccagttgctcccgtaggcggtcattgatgcagatggattcctccaggcgctggcgcaggttccggatttcaccaagatgctcttccagcaggtcagcccctgtgggtttggagttaagctggtacacagaggagcctgaggataggtccccagatacactccctttctgaggcctcatcacatcccacttgccactgctgcccaggtacccaggctctaggattcttcccagttctatggtgccccttggaggagagtgaggctgggcagagttgaggtagtaggaagagtcggcttccaagtcgttgctcagcaatgtagctgtggaagcaggaggaacagtgctggcacctgaatgggcctggttggcctccttgggggtattctggggagttggcaagctgatggggttgctgttggattcggccttagccccctgagatgcactggttgatgatggtttagaagacaacacagcagaatgactcgaatgatggatggaatctgagtgactgggagaagctttcttctcttcatagtgtgtgtactcgctgactatgtccatgtcagagcaggcttccagttcatcagacaggaaagaggtgctgctgggagagcggtgggagtcagacaaggcatggctgctggagggtgtgagggaccgagcatccagcttggcctgcaggacttcaatcactttctccttctcctgcagctccctgctgagcctgagggccagtggctcaagtccagcttgatctttctcacttttatgatccttggtgctgagtttgctggtgagcctctctgtcagctggcttccctgggcgagttgctcccggaagctctgtcccaggtagtagtcaatgtcattgctccttaggagatcctcaaaagattttactgtatcttttgcatgccgggtgataagataacaaatacctctcccttctcgtattttttgccgtaggtaagacagttcccgggcctgatcctgaatcagggaatcatatttcccaggccacgaggctgatctcagctcctcagccagcttctcttctagtccattttttgggagctgggcctccagctgggatactctctggatgagactctccaggtcctttttggcctgaagccctggagagtagaaagccccagtgccatcagacagccacccctcatcctcatcagggacactatgaggtgaagacccctccaaggtgccaacagctctcagcttccggggtctttccagactagacgaataatcacttgtaactgagagggaccggacccggctcttgaggttttgaatgaccttgttggcattctgcagctgggccttcagatctttgatgtcctttcgtaggaccaagatgttttctgactttccatatacccggaactcttcctgcttccctagctggttctccaagggcttcctctcagaggaactagccagtgttgagccccggcgtccctgctcagagcacagcccctccatcaggaccatttccttgaggctgttgtgctcctcacactcaggactggtggtttcctcccgttcagcctcattctcgcttcggccacaagtctcatagcccaggtcctggaggtccacctggatctgcttgctgtcctgcttcaccaaggattcacctgtaagcataactctgtatttctccagctcgttagcctgagcaaagacagtggcttctgatagcagcagcttctcctggagatcttgatagcgttgtttgcattgtgacagctgggagcgcaggtgctgggtggaccctggtaggctaaacgctgactgaggcccagggtcacgaggctgggactggttatccaattggtgggcatccactgtgaaggtagccccaaggtcaaggctctggggtctggggaaaggcctcacagtcacattcccctcctcttggtgttggtgcttcccaggggaaccaaccagttctgtgtttattctttcaatggtgctggtcagatgcacaaggagctctggagtaagtttactattcccttccttgctactcagcacaagttgttctttgaggaggttgatgatattgtgggcattcttcagttttccctggagctttctgaactcagcctgaaggctactctcactcagaccctctttggttaccacagtctcaaccatcacctcgcccttctccttgtcttcctcgatctcccatccatcagacattgcttctcccatctgctctttcagctccgcattctcaaggcaaaggctcagcatggtgttcctgatgtgggacactgaggagaatcctgcttcctcaatttgagcctttagctccttcagttcctcctcagctttcctcttctcttctaagtgctggtggaactcagccctcaggtggagcatttcttcctgaagacacctgttactgtcccctcccatcggagaaggaggggaaaaagatgggttctgggtctccacagttgccagacttttctccaaagccaccttgacaagttgctggtgactatggtgtgcagcctcctcctcaatactgtcagtgaactcagtgcttgtatcttcggtgtcatcccctgcagctgcacctccaatggcggccagggtctccagcctgtttaagcgctccaagcttcttccaagaacttcttctagccgactgcgtaacacctgagccccttccagttccacctgcagagttcggtctctctcagagctctctggatgggcatggaacttcaccagactgctatagagctgtctctctgcttgtaaggcctcattgagccgactccgttcatctactagtccttctagcatcagcagcaactgttgtcttcggtttcctgaaatttcttgaccctgggattctactgaagcaactttttcccgaagaagtaagacttcctgggtcaggcgttccatagctggtatgtcttcaggatcaaccagttgcatttgcaggtcctttatgagatcttctttaatctgtatgttcctggtcagagactccatatcagcagcctgcacctgcagctcttcttcctgcacagccatcatggactgtagagcagaaagttccatctgactttctctttcttttttagccatgagttcaagttcctctttggcattactcagttctttttccagccctgcaactgtgtccaagtctcctaatgtggatctgggtatgctgacatcctctttggcagtcaatgaagtgctatcatctctggaaggtatctgcattgaaccttgatcagtctgttttccaagacggccagtgggggtaacttcagcttgttggttagagatgggtgcttgggacatcagggagtctctccctcctaaatattggcgcagggcctgtaattctgaatttctttccattaaggcttgcaccaacttctctgcagcagcttggctttcctgctccctggtgctcacagactgaagcaggccttgaatctccatttcatgttccagcacttgtttatttcgatcacttagaaggtcctgcagcatcctttcctttcgctgtagacgctggcacagctcctctgctatctcactctgccctggtccaagtttgcagagcagtgttgcactaagatcctccacttctttgttcctatcatgaagagacgtctgtaactgctgaatgatactctcttgttccttctgccaacggctaaatttggtttccatttcttctttcagccactggaggttttgacaggtagtagataactgttccacttccaggcctttggccctcaggagactctccatactttgcatagtagcttcattggaggagaggacatcgcgcagtctctctaagtcatgatctcgctctctcacagcaagacgaagctggcgcagttctttttctttctcttctagagcagagaatttttcatctatagcccgctccagagcaacagctttatcatgtattcgctggcgaagtttctcaagcaacatttcatttgcttcaagggttttgtctgagttatctcgatactgtaggagctcccgaaattcctgaagcaactgctccttgtgactcagactatggtttaggtgctggatgttttgttcctgggttcgaatctcattgtatttttcagcctcccaggcacgaagctgttggctcttattctgcaattcttcttgtagctgctgcaaggcttttcgcaattcctggttatgtttccaagaagcctctttctgctgttcactctcgtgtgctgcagcctctacaaattgcacacattgtttggcatcagccagttggcgctctttctgtcgtaccaccctctggagcttctgtatttcaagttggctgcagaataaagcactctgaagatcaagcagagctacctgttgctgagctggagaagtaccctctgagctgtgaagttgtccaagctggctttggtgcagcatttctcgaagctttgccattgtgtcattttgaccttcaattacctggtacaactcctcagtctcacgttccctgcttttcagagtttccttgaggttctgaattgtaccatcttgcttttgagacgactcctgagcacactttagttcatagctcatttcattaagtttctcttgaagaatcttgttggtggcctctgtttgctggattttttcctggagttctgccaagtgggaatcagatacagactgctgagttatagtggtctcatgtgaattcagcttttgttgtttcagcaactcttcagtcatgggctggacccggagcggcaaataatcttcacagagatcatcccacagctcctgcaggtctgaaagctccaagggataactcacaggtgtcttgtaaaggggtttcaaagacctgttaaggaaaccggaactaactccatctgtcatgctagggccaggcttggctccaggtaggctggatttcactggaatcggaagcctgctccctcgggggctctggatgggcttataatcaagacctttaatcatgctaagagctaattccagcttgtgattacacccatgctgcggagcctgatcatctgaacaacagtcacactttccaagttcctttgcacttctctcagtctcctcatctttctgttgtggagggctagcctggacgcttgcatccaaagattccacagaggaaccaggcgtctcttcctccatgctttctccatctgggggtacctttgtgcttgctaagtcgggtggcccaacctcagacaacgctggttcttcagtgcaaatgctggtcgaccacctgctagaagggccgcaggagatacttctggccacctttcgaggtaccttacaaatggcttcatagtcagaatcagcaacccgcaaagcggcacaaccacggcatctcctgggtcggtttccagggccttctgaaccatggcagctgtgtggctcctggatctgatcctcattctccacccagcactcaaaccctgaataggcgaagtcctcctggagcagtgcagagtatctcgcatcgggtaagacggacatgtcaaccgtcccattccccgccttgatctccgcgccagagtcatcgttattcttccgatacatactggcaatgcagaacttgaggcgatccttctccagtagcagcttttgcaagcgctcaatagaaagcgcttcaatccgggcaataactgtgtcgaatcgatagattcgatcaagcatgaaagcacacttgctgcaagcgaactcggctttgccatcgcgggggacatccttgcccaagacgtgcgaaagcagaacctggagattgagcttggacgccgtgtggaagatccagcgccgctggtttccacacagctctcgggcacagatcctgcaaatctccttcatcttccctcctagcgggtggcaagcttcccgaggcggcggcggcggcggctactgggtgaccactcaatggctcttcgccgcgctctgtctcccgcctcggtggtctccggtcagcatggcacagcccagtggggtccccactctgcaggggcgcgcccctgccccgcgcgccgactccgggtaccagagccgtcagccccgcccctcgggcagggggcgggcgtggaaacgcctaagaggatgctgagtgacagaggcgcaggccgcgctccgaccctgccatgtctctccccagctgtctctcccgccagccgccgcgtcctcaacgtcctccccttttagcagactgggctcccggagcagcagcggccggccgcgcagacgcaaagcctcggggatggaggatc

SEQ ID NO: 8827 - RNA, 7194 nt, Homo sapiens
  source 1..7194: mol_type = other RNA
aagtgtgcagggcactggtgctgctccgaagctcatgaatacctttgctgcctagcacctctgtgccttgggcttcaaggccagggaagctgcacgctgatctcacaagagacactatctttttgaccagcagcttgccctccgcaatctgctgtcttagggcactgtagtcatcaatgtggccaatgacatggcggccatgcttattggcaaaggagccatcagtagcatcaccctctagcttgggaggggtcttcattactggagaagtatccaaacccaagccatttgctctgttgattatgggcgtttctgagccaggagtagaggaagcagagctggggaagaccagagctggggaattcataccaacatcccggactggaggggacacagctgaatctttcagccccttcttggaattgccataaagtgcctcgtagatttgtagctctgactggagggactcaaagagctgctgtttctcttcacactgttgctgcaggagaaccagcttgtgctgcagtctggagtcgttttcctggagggaaagacgttcctccctgaaatgcaagacctcttgctgcttctccctcaagtcttccaaaagctgctgcctttccaccttctggtgctccagctccttttccagctcttgaaggtgggatcgagaggacagcagagcctccctcaggctttctgtttcctgggagtgctctctggaaacatgactcagttgagcctgaagtcttcgattgtcttccctgaggactctgttctcattgcagagctgaggtatggactccaggccctgactgtagaagttagaagtggatccccttccacgagcagtagaggtcagccggtgttccagttgctcccgtaggcggtcattgatgcagatggattcctccaggcgctggcgcaggttccggatttcaccaagatgctcttccagcaggtcagcccctgtgggtttggagttaagctggtacacagaggagcctgaggataggtccccagatacactccctttctgaggcctcatcacatcccacttgccactgctgcccaggtacccaggctctaggattcttcccagttctatggtgccccttggaggagagtgaggctgggcagagttgaggtagtaggaagagtcggcttccaagtcgttgctcagcaatgtagctgtggaagcaggaggaacagtgctggcacctgaatgggcctggttggcctccttgggggtattctggggagttggcaagctgatggggttgctgttggattcggccttagccccctgagatgcactggttgatgatggtttagaagacaacacagcagaatgactcgaatgatggatggaatctgagtgactgggagaagctttcttctcttcatagtgtgtgtactcgctgactatgtccatgtcagagcaggcttccagttcatcagacaggaaagaggtgctgctgggagagcggtgggagtcagacaaggcatggctgctggagggtgtgagggaccgagcatccagcttggcctgcaggacttcaatcactttctccttctcctgcagctccctgctgagcctgagggccagtggctcaagtccagcttgatctttctcacttttatgatccttggtgctgagtttgctggtgagcctctctgtcagctggcttccctgggcgagttgctcccggaagctctgtcccaggtagtagtcaatgtcattgctccttaggagatcctcaaaagattttactgtatcttttgcatgccgggtgataagataacaaatacctctcccttctcgtattttttgccgtaggtaagacagttcccgggcctgatcctgaatcagggaatcatatttcccaggccacgaggctgatctcagctcctcagccagcttctcttctagtccattttttgggagctgggcctccagctgggatactctctggatgagactctccaggtcctttttggcctgaagccctggagagtagaaagccccagtgccatcagacagccacccctcatcctcatcagggacactatgaggtgaagacccctccaaggtgccaacagctctcagcttccggggtctttccagactagacgaataatcacttgtaactgagagggaccggacccggctcttgaggttttgaatgaccttgttggcattctgcagctgggccttcagatctttgatgtcctttcgtaggaccaagatgttttctgactttccatatacccggaactcttcctgcttccctagctggttctccaagggcttcctctcagaggaactagccagtgttgagccccggcgtccctgctcagagcacagcccctccatcaggaccatttccttgaggctgttgtgctcctcacactcaggactggtggtttcctcccgttcagcctcattctcgcttcggccacaagtctcatagcccaggtcctggaggtccacctggatctgcttgctgtcctgcttcaccaaggattcactaagcataactctgtatttctccagctcgttagcctgagcaaagacagtggcttctgatagcagcagcttctcctggagatcttgatagcgttgtttgcattgtgacagctgggagcgcaggtgctgggtggaccctggtaggctaaacgctgactgaggcccagggtcacgaggctgggactggttatccaattggtgggcatccactgtgaaggtagccccaaggtcaaggctctggggtctggggaaaggcctcacagtcacattcccctcctcttggtgttggtgcttcccaggggaaccaaccagttctgtgtttattctttcaatggtgctggtcagatgcacaaggagctctggagtaagtttactattcccttccttgctactcagcacaagttgttctttgaggaggttgatgatattgtgggcattcttcagttttccctggagctttctgaactcagcctgaaggctactctcactcagaccctctttggttaccacagtctcaaccatcacctcgcccttctccttgtcttcctcgatctcccatccatcagacattgcttctcccatctgctctttcagctccgcattctcaaggcaaaggctcagcatggtgttcctgatgtgggacactgaggagaatcctgcttcctcaatttgagcctttagctccttcagttcctcctcagctttcctcttctcttctaagtgctggtggaactcagccctcaggtggagcatttcttcctgaagacacctgttactgtcccctcccatcggagaaggaggggaaaaagatgggttctgggtctccacagttgccagacttttctccaaagccaccttgacaagttgctggtgactatggtgtgcagcctcctcctcaatactgtcagtgaactcagtgcttgtatcttcggtgtcatcccctgcagctgcacctccaatggcggccagggtctccagcctgtttaagcgctccaagcttcttccaagaacttcttctagccgactgcgtaacacctgagccccttccagttccacctgcagagttcggtctctctcagagctctctggatgggcatggaacttcaccagactgctatagagctgtctctctgcttgtaaggcctcattgagccgactccgttcatctactagtccttctagcatcagcagcaactgttgtcttcggtttcctgaaatttcttgaccctgggattctactgaagcaactttttcccgaagaagtaagacttcctgggtcaggcgttccatagctggtatgtcttcaggatcaaccagttgcatttgcaggtcctttatgagatcttctttaatctgtatgttcctggtcagagactccatatcagcagcctgcacctgcagctcttcttcctgcacagccatcatggactgtagagcagaaagttccatctgactttctctttcttttttagccatgagttcaagttcctctttggcattactcagttctttttccagccctgcaactgtgtccaagtctcctaatgtggatctgggtatgctgacatcctctttggcagtcaatgaagtgctatcatctctggaaggtatctgcattgaaccttgatcagtctgttttccaagacggccagtgggggtaacttcagcttgttggttagagatgggtgcttgggacatcagggagtctctccctcctaaatattggcgcagggcctgtaattctgaatttctttccattaaggcttgcaccaacttctctgcagcagcttggctttcctgctccctggtgctcacagactgaagcaggccttgaatctccatttcatgttccagcacttgtttatttcgatcacttagaaggtcctgcagcatcctttcctttcgctgtagacgctggcacagctcctctgctatctcactctgccctggtccaagtttgcagagcagtgttgcactaagatcctccacttctttgttcctatcatgaagagacgtctgtaactgctgaatgatactctcttgttccttctgccaacggctaaatttggtttccatttcttctttcagccactggaggttttgacaggtagtagataactgttccacttccaggcctttggccctcaggagactctccatactttgcatagtagcttcattggaggagaggacatcgcgcagtctctctaagtcatgatctcgctctctcacagcaagacgaagctggcgcagttctttttctttctcttctagagcagagaatttttcatctatagcccgctccagagcaacagctttatcatgtattcgctggcgaagtttctcaagcaacatttcatttgcttcaagggttttgtctgagttatctcgatactgtaggagctcccgaaattcctgaagcaactgctccttgtgactcagactatggtttaggtgctggatgttttgttcctgggttcgaatctcattgtatttttcagcctcccaggcacgaagctgttggctcttattctgcaattcttcttgtagctgctgcaaggcttttcgcaattcctggttatgtttccaagaagcctctttctgctgttcactctcgtgtgctgcagcctctacaaattgcacacattgtttggcatcagccagttggcgctctttctgtcgtaccaccctctggagcttctgtatttcaagttggctgcagaataaagcactctgaagatcaagcagagctacctgttgctgagctggagaagtaccctctgagctgtgaagttgtccaagctggctttggtgcagcatttctcgaagctttgccattgtgtcattttgaccttcaattacctggtacaactcctcagtctcacgttccctgcttttcagagtttccttgaggttctgaattgtaccatcttgcttttgagacgactcctgagcacactttagttcatagctcatttcattaagtttctcttgaagaatcttgttggtggcctctgtttgctggattttttcctggagttctgccaagtgggaatcagatacagactgctgagttatagtggtctcatgtgaattcagcttttgttgtttcagcaactcttcagtcatgggctggacccggagcggcaaataatcttcacagagatcatcccacagctcctgcaggtctgaaagctccaagggataactcacaggtgtcttgtaaaggggtttcaaagacctgttaaggaaaccggaactaactccatctgtcatgctagggccaggcttggctccaggtaggctggatttcactggaatcggaagcctgctccctcgggggctctggatgggcttataatcaagacctttaatcatgctaagagctaattccagcttgtgattacacccatgctgcggagcctgatcatctgaacaacagtcacactttccaagttcctttgcacttctctcagtctcctcatctttctgttgtggagggctagcctggacgcttgcatccaaagattccacagaggaaccaggcgtctcttcctccatgctttctccatctgggggtacctttgtgcttgctaagtcgggtggcccaacctcagacaacgctggttcttcagtgcaaatgctggtcgaccacctgctagaagggccgcaggagatacttctggccacctttcgaggtaccttacaaatggcttcatagtcagaatcagcaacccgcaaagcggcacaaccacggcatctcctgggtcggtttccagggccttctgaaccatggcagctgtgtggctcctggatctgatcctcattctccacccagcactcaaaccctgaataggcgaagtcctcctggagcagtgcagagtatctcgcatcgggtaagacggacatgtcaaccgtcccattccccgccttgatctccgcgccagagtcatcgttattcttccgatacatactggcaatgcagaacttgaggcgatccttctccagtagcagcttttgcaagcgctcaatagaaagcgcttcaatccgggcaataactgtgtcgaatcgatagattcgatcaagcatgaaagcacacttgctgcaagcgaactcggctttgccatcgcgggggacatccttgcccaagacgtgcgaaagcagaacctggagattgagcttggacgccgtgtggaagatccagcgccgctggtttccacacagctctcgggcacagatcctgcaaatctccttcatcttccctcctagcgggtggcaagcttcccgaggcggcggcggcggcggctactgggtgaccactcaatggctcttcgccgcgctctgtctcccgcctcggtggtctccggtcagcatggcacagcccagtggggtccccactctgcaggggcgcgcccctgccccgcgcgccgactccgggtaccagagccgtcagccccgcccctcgggcagggggcgggcgtggaaacgcctaagaggatgctgagtgacagaggcgcaggccgcgctccgaccctgccatgtctctccccagctgtctctcccgccagccgccgcgtcctcaacgtcctccccttttagcagactgggctcccggagcagcagcggccggccgcgcagacgcaaagcctcggggatggaggatc

SEQ ID NO: 8828 - RNA, 7383 nt, Homo sapiens
  source 1..7383: mol_type = other RNA
aagtgtgcagggcactggtgctgctccgaagctcatgaatacctttgctgcctagcacctctgtgccttgggcttcaaggccagggaagctgcacgctgatctcacaagagacactatctttttgaccagcagcttgccctccgcaatctgctgtcttagggcactgtagtcatcaatgtggccaatgacatggcggccatgcttattggcaaaggagccatcagtagcatcaccctctagcttgggaggggtcttcattactggagaagtatccaaacccaagccatttgctctgttgattatgggcgtttctgagccaggagtagaggaagcagagctggggaagaccagagctggggaattcataccaacatcccggactggaggggacacagctgaatctttcagccccttcttggaattgccataaagtgcctcgtagatttgtagctctgactggagggactcaaagagctgctgtttctcttcacactgttgctgcaggagaaccagcttgtgctgcagtctggagtcgttttcctggagggaaagacgttcctccctgaaatgcaagacctcttgctgcttctccctcaagtcttccaaaagctgctgcctttccaccttctggtgctccagctccttttccagctcttgaaggtgggatcgagaggacagcagagcctccctcaggctttctgtttcctgggagtgctctctggaaacatgactcagttgagcctgaagtcttcgattgtcttccctgaggactctgttctcattgcagagctgaggtatggactccaggccctgactgtagaagttagaagtggatccccttccacgagcagtagaggtcagccggtgttccagttgctcccgtaggcggtcattgatgcagatggattcctccaggcgctggcgcaggttccggatttcaccaagatgctcttccagcaggtcagcccctgtgggtttggagttaagctggtacacagaggagcctgaggataggtccccagatacactccctttctgaggcctcatcacatcccacttgccactgctgcccaggtacccaggctctaggattcttcccagttctatggtgccccttggaggagagtgaggctgggcagagttgaggtagtaggaagagtcggcttccaagtcgttgctcagcaatgtagctgtggaagcaggaggaacagtgctggcactttctcccaactgcttctgcagcatctgtagctcctgctgagcctcagccaaggagaccactggtgtctcacagcagccaaggaggagagggccagtggggctgaaaggcaggaagctggatggagctgagggcaatggtgcctgaggaaggctagccagcttgggtatggagtgaaaatgaaagcctgaatgggcctggttggcctccttgggggtattctggggagttggcaagctgatggggttgctgttggattcggccttagccccctgagatgcactggttgatgatggtttagaagacaacacagcagaatgactcgaatgatggatggaatctgagtgactgggagaagctttcttctcttcatagtgtgtgtactcgctgactatgtccatgtcagagcaggcttccagttcatcagacaggaaagaggtgctgctgggagagcggtgggagtcagacaaggcatggctgctggagggtgtgagggaccgagcatccagcttggcctgcaggacttcaatcactttctccttctcctgcagctccctgctgagcctgagggccagtggctcaagtccagcttgatctttctcacttttatgatccttggtgctgagtttgctggtgagcctctctgtcagctggcttccctgggcgagttgctcccggaagctctgtcccaggtagtagtcaatgtcattgctccttaggagatcctcaaaagattttactgtatcttttgcatgccgggtgataagataacaaatacctctcccttctcgtattttttgccgtaggtaagacagttcccgggcctgatcctgaatcagggaatcatatttcccaggccacgaggctgatctcagctcctcagccagcttctcttctagtccattttttgggagctgggcctccagctgggatactctctggatgagactctccaggtcctttttggcctgaagccctggagagtagaaagccccagtgccatcagacagccacccctcatcctcatcagggacactatgaggtgaagacccctccaaggtgccaacagctctcagcttccggggtctttccagactagacgaataatcacttgtaactgagagggaccggacccggctcttgaggttttgaatgaccttgttggcattctgcagctgggccttcagatctttgatgtcctttcgtaggaccaagatgttttctgactttccatatacccggaactcttcctgcttccctagctggttctccaagggcttcctctcagaggaactagccagtgttgagccccggcgtccctgctcagagcacagcccctccatcaggaccatttccttgaggctgttgtgctcctcacactcaggactggtggtttcctcccgttcagcctcattctcgcttcggccacaagtctcatagcccaggtcctggaggtccacctggatctgcttgctgtcctgcttcaccaaggattcacctgtaagcataactctgtatttctccagctcgttagcctgagcaaagacagtggcttctgatagcagcagcttctcctggagatcttgatagcgttgtttgcattgtgacagctgggagcgcaggtgctgggtggaccctggtaggctaaacgctgactgaggcccagggtcacgaggctgggactggttatccaattggtgggcatccactgtgaaggtagccccaaggtcaaggctctggggtctggggaaaggcctcacagtcacattcccctcctcttggtgttggtgcttcccaggggaaccaaccagttctgtgtttattctttcaatggtgctggtcagatgcacaaggagctctggagtaagtttactattcccttccttgctactcagcacaagttgttctttgaggaggttgatgatattgtgggcattcttcagttttccctggagctttctgaactcagcctgaaggctactctcactcagaccctctttggttaccacagtctcaaccatcacctcgcccttctccttgtcttcctcgatctcccatccatcagacattgcttctcccatctgctctttcagctccgcattctcaaggcaaaggctcagcatggtgttcctgatgtgggacactgaggagaatcctgcttcctcaatttgagcctttagctccttcagttcctcctcagctttcctcttctcttctaagtgctggtggaactcagccctcaggtggagcatttcttcctgaagacacctgttactgtcccctcccatcggagaaggaggggaaaaagatgggttctgggtctccacagttgccagacttttctccaaagccaccttgacaagttgctggtgactatggtgtgcagcctcctcctcaatactgtcagtgaactcagtgcttgtatcttcggtgtcatcccctgcagctgcacctccaatggcggccagggtctccagcctgtttaagcgctccaagcttcttccaagaacttcttctagccgactgcgtaacacctgagccccttccagttccacctgcagagttcggtctctctcagagctctctggatgggcatggaacttcaccagactgctatagagctgtctctctgcttgtaaggcctcattgagccgactccgttcatctactagtccttctagcatcagcagcaactgttgtcttcggtttcctgaaatttcttgaccctgggattctactgaagcaactttttcccgaagaagtaagacttcctgggtcaggcgttccatagctggtatgtcttcaggatcaaccagttgcatttgcaggtcctttatgagatcttctttaatctgtatgttcctggtcagagactccatatcagcagcctgcacctgcagctcttcttcctgcacagccatcatggactgtagagcagaaagttccatctgactttctctttcttttttagccatgagttcaagttcctctttggcattactcagttctttttccagccctgcaactgtgtccaagtctcctaatgtggatctgggtatgctgacatcctctttggcagtcaatgaagtgctatcatctctggaaggtatctgcattgaaccttgatcagtctgttttccaagacggccagtgggggtaacttcagcttgttggttagagatgggtgcttgggacatcagggagtctctccctcctaaatattggcgcagggcctgtaattctgaatttctttccattaaggcttgcaccaacttctctgcagcagcttggctttcctgctccctggtgctcacagactgaagcaggccttgaatctccatttcatgttccagcacttgtttatttcgatcacttagaaggtcctgcagcatcctttcctttcgctgtagacgctggcacagctcctctgctatctcactctgccctggtccaagtttgcagagcagtgttgcactaagatcctccacttctttgttcctatcatgaagagacgtctgtaactgctgaatgatactctcttgttccttctgccaacggctaaatttggtttccatttcttctttcagccactggaggttttgacaggtagtagataactgttccacttccaggcctttggccctcaggagactctccatactttgcatagtagcttcattggaggagaggacatcgcgcagtctctctaagtcatgatctcgctctctcacagcaagacgaagctggcgcagttctttttctttctcttctagagcagagaatttttcatctatagcccgctccagagcaacagctttatcatgtattcgctggcgaagtttctcaagcaacatttcatttgcttcaagggttttgtctgagttatctcgatactgtaggagctcccgaaattcctgaagcaactgctccttgtgactcagactatggtttaggtgctggatgttttgttcctgggttcgaatctcattgtatttttcagcctcccaggcacgaagctgttggctcttattctgcaattcttcttgtagctgctgcaaggcttttcgcaattcctggttatgtttccaagaagcctctttctgctgttcactctcgtgtgctgcagcctctacaaattgcacacattgtttggcatcagccagttggcgctctttctgtcgtaccaccctctggagcttctgtatttcaagttggctgcagaataaagcactctgaagatcaagcagagctacctgttgctgagctggagaagtaccctctgagctgtgaagttgtccaagctggctttggtgcagcatttctcgaagctttgccattgtgtcattttgaccttcaattacctggtacaactcctcagtctcacgttccctgcttttcagagtttccttgaggttctgaattgtaccatcttgcttttgagacgactcctgagcacactttagttcatagctcatttcattaagtttctcttgaagaatcttgttggtggcctctgtttgctggattttttcctggagttctgccaagtgggaatcagatacagactgctgagttatagtggtctcatgtgaattcagcttttgttgtttcagcaactcttcagtcatgggctggacccggagcggcaaataatcttcacagagatcatcccacagctcctgcaggtctgaaagctccaagggataactcacaggtgtcttgtaaaggggtttcaaagacctgttaaggaaaccggaactaactccatctgtcatgctagggccaggcttggctccaggtaggctggatttcactggaatcggaagcctgctccctcgggggctctggatgggcttataatcaagacctttaatcatgctaagagctaattccagcttgtgattacacccatgctgcggagcctgatcatctgaacaacagtcacactttccaagttcctttgcacttctctcagtctcctcatctttctgttgtggagggctagcctggacgcttgcatccaaagattccacagaggaaccaggcgtctcttcctccatgctttctccatctgggggtacctttgtgcttgctaagtcgggtggcccaacctcagacaacgctggttcttcagtgcaaatgctggtcgaccacctgctagaagggccgcaggagatacttctggccacctttcgaggtaccttacaaatggcttcatagtcagaatcagcaacccgcaaagcggcacaaccacggcatctcctgggtcggtttccagggccttctgaaccatggcagctgtgtggctcctggatctgatcctcattctccacccagcactcaaaccctgaataggcgaagtcctcctggagcagtgcagagtatctcgcatcgggtaagacggacatgtcaaccgtcccattccccgccttgatctccgcgccagagtcatcgttattcttccgatacatactggcaatgcagaacttgaggcgatccttctccagtagcagcttttgcaagcgctcaatagaaagcgcttcaatccgggcaataactgtgtcgaatcgatagattcgatcaagcatgaaagcacacttgctgcaagcgaactcggctttgccatcgcgggggacatccttgcccaagacgtgcgaaagcagaacctggagattgagcttggacgccgtgtggaagatccagcgccgctggtttccacacagctctcgggcacagatcctgcaaatctccttcatcttccctcctagcgggtggcaagcttcccgaggcggcggcggcggcggctactgggtgaccactcaatggctcttcgccgcgctctgtctcccgcctcggtggtctccggtcagcatggcacagcccagtggggtccccactctgcaggggcgcgcccctgccccgcgcgccgactccgggtaccagagccgtcagccccgcccctcgggcagggggcgggcgtggaaacgcctaagaggatgctgagtgacagaggcgcaggccgcgctccgaccctgccatgtctctccccagctgtctctcccgccagccgccgcgtcctcaacgtcctccccttttagcagactgggctcccggagcagcagcggccggccgcgcagacgcaaagcctcggggatggaggatc

SEQ ID NO: 8829 - RNA, 7184 nt, Homo sapiens
  source 1..7184: mol_type = other RNA
aagtgtgcagggcactggtgctgctccgaagctcatgaatacctttgctgcctagcacctctgtgccttgggcttcaaggccagggaagctgcacgctgatctcacaagagacactatctttttgaccagcagcttgccctccgcaatctgctgtcttagggcactgtagtcatcaatgtggccaatgacatggcggccatgcttattggcaaaggagccatcagtagcatcaccctctagcttgggaggggtcttcattactggagaagtatccaaacccaagccttggaggagcagctgcttgtttccagggtcagtgctggctgggaagttctggttaatggaggaggggctgaggctggctttgccagcaccgctctccagctgctgttgcagctgcagtcgcagacaattgttcccctgaatgctctgctccagctgccctctcagagctcgtacctctgccaccaggtggctcaggtcactgctcaaagggatttggtgacaggcatccaggctgtaagctttcagccccttcttggaattgccataaagtgcctcgtagatttgtagctctgactggagggactcaaagagctgctgtttctcttcacactgttgctgcaggagaaccagcttgtgctgcagtctggagtcgttttcctggagggaaagacgttcctccctgaaatgcaagacctcttgctgcttctccctcaagtcttccaaaagctgctgcctttccaccttctggtgctccagctccttttccagctcttgaaggtgggatcgagaggacagcagagcctccctcaggctttctgtttcctgggagtgctctctggaaacatgactcagttgagcctgaagtcttcgattgtcttccctgaggactctgttctcattgcagagctgaggtatggactccaggccctgactgtagaagttagaagtggatccccttccacgagcagtagaggtcagccggtgttccagttgctcccgtaggcggtcattgatgcagatggattcctccaggcgctggcgcaggttccggatttcaccaagatgctcttccagcaggtcagcccctgtgggtttggagttaagctggtacacagaggagcctgaggataggtccccagatacactccctttctgaggcctcatcacatcccacttgccactgctgcccaggtacccaggctctaggattcttcccagttctatggtgccccttggaggagagtgaggctgggcagagttgaggtagtaggaagagtcggcttccaagtcgttgctcagcaatgtagctgtggaagcaggaggaacagtgctggcactttctcccaactgcttctgcagcatctgtagctcctgctgagcctcagccaaggagaccactggtgtctcacagcagccaaggaggagagggccagtggggctgaaaggcaggaagctggatggagctgagggcaatggtgcctgaggaaggctagccagcttgggtatggagtgaaaatgaaagcctgaatgggcctggttggcctccttgggggtattctggggagttggcaagctgatggggttgctgttggattcggccttagccccctgagatgcactggttgatgatggtttagaagacaacacagcagaatgactcgaatgatggatggaatctgagtgactgggagaagctttcttctcttcatagtgtgtgtactcgctgactatgtccatgtcagagcaggcttccagttcatcagacaggaaagaggtgctgctgggagagcggtgggagtcagacaaggcatggctgctggagggtgtgagggaccgagcatccagcttggcctgcaggacttcaatcactttctccttctcctgcagctccctgctgagcctgagggccagtggctcaagtccagcttgatctttctcacttttatgatccttggtgctgagtttgctggtgagcctctctgtcagctggcttccctgggcgagttgctcccggaagctctgtcccaggtagtagtcaatgtcattgctccttaggagatcctcaaaagattttactgtatcttttgcatgccgggtgataagataacaaatacctctcccttctcgtattttttgccgtaggtaagacagttcccgggcctgatcctgaatcagggaatcatatttcccaggccacgaggctgatctcagctcctcagccagcttctcttctagtccattttttgggagctgggcctccagctgggatactctctggatgagactctccaggtcctttttggcctgaagccctggagagtagaaagccccagtgccatcagacagccacccctcatcctcatcagggacactatgaggtgaagacccctccaaggtgccaacagctctcagcttccggggtctttccagactagacgaataatcacttgtaactgagagggaccggacccggctcttgaggttttgaatgaccttgttggcattctgcagctgggccttcagatctttgatgtcctttcgtaggaccaagatgttttctgactttccatatacccggaactcttcctgcttccctagctggttctccaagggcttcctctcagaggaactagccagtgttgagccccggcgtccctgctcagagcacagcccctccatcaggaccatttccttgaggctgttgtgctcctcacactcaggactggtggtttcctcccgttcagcctcattctcgcttcggccacaagtctcatagcccaggtcctggaggtccacctggatctgcttgctgtcctgcttcaccaaggattcacctgtaagcataactctgtatttctccagctcgttagcctgagcaaagacagtggcttctgatagcagcagcttctcctggagatcttgatagcgttgtttgcattgtgacagctgggagcgcaggtgctgggtggaccctggtaggctaaacgctgactgaggcccagggtcacgaggctgggactggttatccaattggtgggcatccactgtgaaggtagccccaaggtcaaggctctggggtctggggaaaggcctcacagtcacattcccctcctcttggtgttggtgcttcccaggggaaccaaccagttctgtgtttattctttcaatggtgctggtcagatgcacaaggagctctggagtaagtttactattcccttccttgctactcagcacaagttgttctttgaggaggttgatgatattgtgggcattcttcagttttccctggagctttctgaactcagcctgaaggctactctcactcagaccctctttggttaccacagtctcaaccatcacctcgcccttctccttgtcttcctcgatctcccatccatcagacattgcttctcccatctgctctttcagctccgcattctcaaggcaaaggctcagcatggtgttcctgatgtgggacactgaggagaatcctgcttcctcaatttgagcctttagctccttcagttcctcctcagctttcctcttctcttctaagtgctggtggaactcagccctcaggtggagcatttcttcctgaagacacctgttactgtcccctcccatcggagaaggaggggaaaaagatgggttctgggtctccacagttgccagacttttctccaaagccaccttgacaagttgctggtgactatggtgtgcagcctcctcctcaatactgtcagtgaactcagtgcttgtatcttcggtgtcatcccctgcagctgcacctccaatggcggccagggtctccagcctgtttaagcgctccaagcttcttccaagaacttcttctagccgactgcgtaacacctgagccccttccagttccacctgcagagttcggtctctctcagagctctctggatgggcatggaacttcaccagactgctatagagctgtctctctgcttgtaaggcctcattgagccgactccgttcatctactagtccttctagcatcagcagcaactgttgtcttcggtttcctgaaatttcttgaccctgggattctactgaagcaactttttcccgaagaagtaagacttcctgggtcaggcgttccatagctggtatgtcttcaggatcaaccagttgcatttgcaggtcctttatgagatcttctttaatctgtatgttcctggtcagagactccatatcagcagcctgcacctgcagctcttcttcctgcacagccatcatggactgtagagcagaaagttccatctgactttctctttcttttttagccatgagttcaagttcctctttggcattactcagttctttttccagccctgcaactgtgtccaagtctcctaatgtggatctgggtatgctgacatcctctttggcagtcaatgaagtgctatcatctctggaaggtatctgcattgaaccttgatcagtctgttttccaagacggccagtgggggtaacttcagcttgttggttagagatgggtgcttgggacatcagggagtctctccctcctaaatattggcgcagggcctgtaattctgaatttctttccattaaggcttgcaccaacttctctgcagcagcttggctttcctgctccctggtgctcacagactgaagcaggccttgaatctccatttcatgttccagcacttgtttatttcgatcacttagaaggtcctgcagcatcctttcctttcgctgtagacgctggcacagctcctctgctatctcactctgccctggtccaagtttgcagagcagtgttgcactaagatcctccacttctttgttcctatcatgaagagacgtctgtaactgctgaatgatactctcttgttccttctgccaacggctaaatttggtttccatttcttctttcagccactggaggttttgacaggtagtagataactgttccacttccaggcctttggccctcaggagactctccatactttgcatagtagcttcattggaggagaggacatcgcgcagtctctctaagtcatgatctcgctctctcacagcaagacgaagctggcgcagttctttttctttctcttctagagcagagaatttttcatctatagcccgctccagagcaacagctttatcatgtattcgctggcgaagtttctcaagcaacatttcatttgcttcaagggttttgtctgagttatctcgatactgtaggagctcccgaaattcctgaagcaactgctccttgtgactcagactatggtttaggtgctggatgttttgttcctgggttcgaatctcattgtatttttcagcctcccaggcacgaagctgttggctcttattctgcaattcttcttgtagctgctgcaaggcttttcgcaattcctggttatgtttccaagaagcctctttctgctgttcactctcgtgtgctgcagcctctacaaattgcacacattgtttggcatcagccagttggcgctctttctgtcgtaccaccctctggagcttctgtatttcaagttggctgcagaataaagcactctgaagatcaagcagagctacctgttgctgagctggagaagtaccctctgagctgtgaagttgtccaagctggctttggtgcagcatttctcgaagctttgccattgtgtcattttgaccttcaattacctggtacaactcctcagtctcacgttccctgcttttcagagtttccttgaggttctgaattgtaccatcttgcttttgagacgactcctgagcacactttagttcatagctcatttcattaagtttctcttgaagaatcttgttggtggcctctgtttgctggattttttcctggagttctgccaagtgggaatcagatacagactgctgagttatagtggtctcatgtgaattcagcttttgttgtttcagcaactcttcagtcatgggctgcacttccatgctagttggctcctccaacagatgtagcagttgttgtttctcccgagatagctgttctacaagcctctcctgggcagccaggctctgattcagttcttcaattctcttgtccctctgggccagggcctcagtgtattggtcgggcttgacctggtctcctggtacatcttcccagtttttggtgactcccttcagtttctctgagagctccaggttacactccttctctgcttccaccagagctgccatccgcgcagcttcattctttgctagcctggattcctcctgcagaagctggatcttattctccaagagctcataaacatgctccgtctcctgctgtcgctcctcaaactggcgtcggagctcagcttcattctgactgttgagattctccacatcagcccatgttttatccagatgctgtttcttgtcctggagttctcgtttcaagctctccacttcaaccttcagctcaatgttccgcttgtagatgtcctcccggctggcctcatacttctgttgcatgcgctcctccaggaagtagatgcgcagcttgaggctgaagttctccttcttcaggtcattgaggtgcttctcaaagtctcgaagagcctgggtctgtacctgagggggtttctcaaatgctctcaaggaatatgtctgcacaaacgggaccttttcaccacttctccagatctgtgactgcactggagggcctcgatctttagtgtcactaagaaaagctgctgtgtgactcgttctgggtaccatctccccatcatcctctgcaaaataatctctcatccagggtgtggccgccgcagctgcttcttcctcctcggccgctgctgcccagctcccggctggctccgggcgccgtctttcccggctcggggtctgccgtggggactgaggggttcgcgtcgcgtccccggaccggtaaggcgtgtagtgagcccggcgggacgcgcgacagcagcagccaaagtcgcatcggcggcggcagcaggacccgctgtctgtgcccttcatggatttcctgggcctggccaccccagtcctagctacggttcctgcttgttttcctggtgttttccgggactgccagggcgcatcctctgggcctggctgagcatccccgtcagttccctgggcctcctccgcggctgcctctgccacctgctccgcccagatt

SEQ ID NO: 8830 - RNA, 7088 nt, Homo sapiens
  source 1..7088: mol_type = other RNA
aagtgtgcagggcactggtgctgctccgaagctcatgaatacctttgctgcctagcacctctgtgccttgggcttcaaggccagggaagctgcacgctgatctcacaagagacactatctttttgaccagcagcttgccctccgcaatctgctgtcttagggcactgtagtcatcaatgtggccaatgacatggcggccatgcttattggcaaaggagccatcagtagcatcaccctctagcttgggaggggtcttcattactggagaagtatccaaacccaagcctttcagccccttcttggaattgccataaagtgcctcgtagatttgtagctctgactggagggactcaaagagctgctgtttctcttcacactgttgctgcaggagaaccagcttgtgctgcagtctggagtcgttttcctggagggaaagacgttcctccctgaaatgcaagacctcttgctgcttctccctcaagtcttccaaaagctgctgcctttccaccttctggtgctccagctccttttccagctcttgaaggtgggatcgagaggacagcagagcctccctcaggctttctgtttcctgggagtgctctctggaaacatgactcagttgagcctgaagtcttcgattgtcttccctgaggactctgttctcattgcagagctgaggtatggactccaggccctgactgtagaagttagaagtggatccccttccacgagcagtagaggtcagccggtgttccagttgctcccgtaggcggtcattgatgcagatggattcctccaggcgctggcgcaggttccggatttcaccaagatgctcttccagcaggtcagcccctgtgggtttggagttaagctggtacacagaggagcctgaggataggtccccagatacactccctttctgaggcctcatcacatcccacttgccactgctgcccaggtacccaggctctaggattcttcccagttctatggtgccccttggaggagagtgaggctgggcagagttgaggtagtaggaagagtcggcttccaagtcgttgctcagcaatgtagctgtggaagcaggaggaacagtgctggcactttctcccaactgcttctgcagcatctgtagctcctgctgagcctcagccaaggagaccactggtgtctcacagcagccaaggaggagagggccagtggggctgaaaggcaggaagctggatggagctgagggcaatggtgcctgaggaaggctagccagcttgggtatggagtgaaaatgaaagcctgaatgggcctggttggcctccttgggggtattctggggagttggcaagctgatggggttgctgttggattcggccttagccccctgagatgcactggttgatgatggtttagaagacaacacagcagaatgactcgaatgatggatggaatctgagtgactgggagaagctttcttctcttcatagtgtgtgtactcgctgactatgtccatgtcagagcaggcttccagttcatcagacaggaaagaggtgctgctgggagagcggtgggagtcagacaaggcatggctgctggagggtgtgagggaccgagcatccagcttggcctgcaggacttcaatcactttctccttctcctgcagctccctgctgagcctgagggccagtggctcaagtccagcttgatctttctcacttttatgatccttggtgctgagtttgctggtgagcctctctgtcagctggcttccctgggcgagttgctcccggaagctctgtcccaggtagtagtcaatgtcattgctccttaggagatcctcaaaagattttactgtatcttttgcatgccgggtgataagataacaaatacctctcccttctcgtattttttgccgtaggtaagacagttcccgggcctgatcctgaatcagggaatcatatttcccaggccacgaggctgatctcagctcctcagccagcttctcttctagtccattttttgggagctgggcctccagctgggatactctctggatgagactctccaggtcctttttggcctgaagccctggagagtagaaagccccagtgccatcagacagccacccctcatcctcatcagggacactatgaggtgaagacccctccaaggtgccaacagctctcagcttccggggtctttccagactagacgaataatcacttgtaactgagagggaccggacccggctcttgaggttttgaatgaccttgttggcattctgcagctgggccttcagatctttgatgtcctttcgtaggaccaagatgttttctgactttccatatacccggaactcttcctgcttccctagctggttctccaagggcttcctctcagaggaactagccagtgttgagccccggcgtccctgctcagagcacagcccctccatcaggaccatttccttgaggctgttgtgctcctcacactcaggactggtggtttcctcccgttcagcctcattctcgcttcggccacaagtctcatagcccaggtcctggaggtccacctggatctgcttgctgtcctgcttcaccaaggattcacctgtaagcataactctgtatttctccagctcgttagcctgagcaaagacagtggcttctgatagcagcagcttctcctggagatcttgatagcgttgtttgcattgtgacagctgggagcgcaggtgctgggtggaccctggtaggctaaacgctgactgaggcccagggtcacgaggctgggactggttatccaattggtgggcatccactgtgaaggtagccccaaggtcaaggctctggggtctggggaaaggcctcacagtcacattcccctcctcttggtgttggtgcttcccaggggaaccaaccagttctgtgtttattctttcaatggtgctggtcagatgcacaaggagctctggagtaagtttactattcccttccttgctactcagcacaagttgttctttgaggaggttgatgatattgtgggcattcttcagttttccctggagctttctgaactcagcctgaaggctactctcactcagaccctctttggttaccacagtctcaaccatcacctcgcccttctccttgtcttcctcgatctcccatccatcagacattgcttctcccatctgctctttcagctccgcattctcaaggcaaaggctcagcatggtgttcctgatgtgggacactgaggagaatcctgcttcctcaatttgagcctttagctccttcagttcctcctcagctttcctcttctcttctaagtgctggtggaactcagccctcaggtggagcatttcttcctgaagacacctgttactgtcccctcccatcggagaaggaggggaaaaagatgggttctgggtctccacagttgccagacttttctccaaagccaccttgacaagttgctggtgactatggtgtgcagcctcctcctcaatactgtcagtgaactcagtgcttgtatcttcggtgtcatcccctgcagctgcacctccaatggcggccagggtctccagcctgtttaagcgctccaagcttcttccaagaacttcttctagccgactgcgtaacacctgagccccttccagttccacctgcagagttcggtctctctcagagctctctggatgggcatggaacttcaccagactgctatagagctgtctctctgcttgtaaggcctcattgagccgactccgttcatctactagtccttctagcatcagcagcaactgttgtcttcggtttcctgaaatttcttgaccctgggattctactgaagcaactttttcccgaagaagtaagacttcctgggtcaggcgttccatagctggtatgtcttcaggatcaaccagttgcatttgcaggtcctttatgagatcttctttaatctgtatgttcctggtcagagactccatatcagcagcctgcacctgcagctcttcttcctgcacagccatcatggactgtagagcagaaagttccatctgactttctctttcttttttagccatgagttcaagttcctctttggcattactcagttctttttccagccctgcaactgtgtccaagtctcctaatgtggatctgggtatgctgacatcctctttggcagtcaatgaagtgctatcatctctggaaggtatctgcattgaaccttgatcagtctgttttccaagacggccagtgggggtaacttcagcttgttggttagagatgggtgcttgggacatcagggagtctctccctcctaaatattggcgcagggcctgtaattctgaatttctttccattaaggcttgcaccaacttctctgcagcagcttggctttcctgctccctggtgctcacagactgaagcaggccttgaatctccatttcatgttccagcacttgtttatttcgatcacttagaaggtcctgcagcatcctttcctttcgctgtagacgctggcacagctcctctgctatctcactctgccctggtccaagtttgcagagcagtgttgcactaagatcctccacttctttgttcctatcatgaagagacgtctgtaactgctgaatgatactctcttgttccttctgccaacggctaaatttggtttccatttcttctttcagccactggaggttttgacaggtagtagataactgttccacttccaggcctttggccctcaggagactctccatactttgcatagtagcttcattggaggagaggacatcgcgcagtctctctaagtcatgatctcgctctctcacagcaagacgaagctggcgcagttctttttctttctcttctagagcagagaatttttcatctatagcccgctccagagcaacagctttatcatgtattcgctggcgaagtttctcaagcaacatttcatttgcttcaagggttttgtctgagttatctcgatactgtaggagctcccgaaattcctgaagcaactgctccttgtgactcagactatggtttaggtgctggatgttttgttcctgggttcgaatctcattgtatttttcagcctcccaggcacgaagctgttggctcttattctgcaattcttcttgtagctgctgcaaggcttttcgcaattcctggttatgtttccaagaagcctctttctgctgttcactctcgtgtgctgcagcctctacaaattgcacacattgtttggcatcagccagttggcgctctttctgtcgtaccaccctctggagcttctgtatttcaagttggctgcagaataaagcactctgaagatcaagcagagctacctgttgctgagctggagaagtaccctctgagctgtgaagttgtccaagctggctttggtgcagcatttctcgaagctttgccattgtgtcattttgaccttcaattacctggtacaactcctcagtctcacgttccctgcttttcagagtttccttgaggttctgaattgtaccatcttgcttttgagacgactcctgagcacactttagttcatagctcatttcattaagtttctcttgaagaatcttgttggtggcctctgtttgctggattttttcctggagttctgccaagtgggaatcagatacagactgctgagttatagtggtctcatgtgaattcagcttttgttgtttcagcaactcttcagtcatgggctgcacttccatgctagttggctcctccaacagatgtagcagttgttgtttctcccgagatagctgttctacaagcctctcctgggcagccaggctctgattcagttcttcaattctcttgtccctctgggccagggcctcagtgtattggtcgggcttgacctggtctcctggtacatcttcccagtttttggtgactcccttcagtttctctgagagctccaggttacactccttctctgcttccaccagagctgccatccgcgcagcttcattctttgctagcctggattcctcctgcagaagctggatcttattctccaagagctcataaacatgctccgtctcctgctgtcgctcctcaaactggcgtcggagctcagcttcattctgactgttgagattctccacatcagcccatgttttatccagatgctgtttcttgtcctggagttctcgtttcaagctctccacttcaaccttcagctcaatgttccgcttgtagatgtcctcccggctggcctcatacttctgttgcatgcgctcctccaggaagtagatgcgcagcttgaggctgaagttctccttcttcaggtcattgaggtgcttctcaaagtctcgaagagcctgggtctgtacctgagggggtttctcaaatgctctcaaggaatatgtctgcacaaacgggaccttttcaccacttctccagatctgtgactgcactggagggcctcgatctttagtgtcactaagaaaagctgctgtgtgactcgttctgggtaccatctccccatcatcctctgcaaaataatctctcatccagggtgtggccgccgcagctgcttcttcctcctcggccgctgctgcccagctcccggctggctccgggcgccgtctttcccggctcggggtctgccgtggggactgaggggttcgcgtcgcgtccccggaccggtaaggcgtgtagtgagcccggcgggacgcgcgacagcagcagccaaagtcgcatcggcggcggcagcaggacccgctgtctgtgcccttcatggatttcctgggcctggccaccccagtcctagctacggttcctgcttgttttcctggtgttttccgggactgccagggcgcatcctctgggcctggctgagcatccccgtcagttccctgggcctcctccgcggctgcctctgccacctgctccgcccagattgctttggtccttctcccgcagacacactcagctgcccttcatcctctgtcgtctccccattctctctccacccactgcctcattcccagatcccacgccgtttcttcctttctatccgctccaatgtcaccttctctttatttc

SEQ ID NO: 8831 - RNA, 6915 nt, Homo sapiens
  source 1..6915: mol_type = other RNA
aagtgtgcagggcactggtgctgctccgaagctcatgaatacctttgctgcctagcacctctgtgccttgggcttcaaggccagggaagctgcacgctgatctcacaagagacactatctttttgaccagcagcttgccctccgcaatctgctgtcttagggcactgtagtcatcaatgtggccaatgacatggcggccatgcttattggcaaaggagccatcagtagcatcaccctctagcttgggaggggtcttcattactggagaagtatccaaacccaagcctttcagccccttcttggaattgccataaagtgcctcgtagatttgtagctctgactggagggactcaaagagctgctgtttctcttcacactgttgctgcaggagaaccagcttgtgctgcagtctggagtcgttttcctggagggaaagacgttcctccctgaaatgcaagacctcttgctgcttctccctcaagtcttccaaaagctgctgcctttccaccttctggtgctccagctccttttccagctcttgaaggtgggatcgagaggacagcagagcctccctcaggctttctgtttcctgggagtgctctctggaaacatgactcagttgagcctgaagtcttcgattgtcttccctgaggactctgttctcattgcagagctgaggtatggactccaggccctgactgtagaagttagaagtggatccccttccacgagcagtagaggtcagccggtgttccagttgctcccgtaggcggtcattgatgcagatggattcctccaggcgctggcgcaggttccggatttcaccaagatgctcttccagcaggtcagcccctgtgggtttggagttaagctggtacacagaggagcctgaggataggtccccagatacactccctttctgaggcctcatcacatcccacttgccactgctgcccaggtacccaggctctaggattcttcccagttctatggtgccccttggaggagagtgaggctgggcagagttgaggtagtaggaagagtcggcttccaagtcgttgctcagcaatgtagctgtggaagcaggaggaacagtgctggcactttctcccaactgcttctgcagcatctgtagctcctgctgagcctcagccaaggagaccactggtgtctcacagcagccaaggaggagagggccagtggggctgaaaggcaggaagctggatggagctgagggcaatggtgcctgaggaaggctagccagcttgggtatggagtgaaaatgaaagcctgaatgggcctggttggcctccttgggggtattctggggagttggcaagctgatggggttgctgttggattcggccttagccccctgagatgcactggttgatgatggtttagaagacaacacagcagaatgactcgaatgatggatggaatctgagtgactgggagaagctttcttctcttcatagtgtgtgtactcgctgactatgtccatgtcagagcaggcttccagttcatcagacaggaaagaggtgctgctgggagagcggtgggagtcagacaaggcatggctgctggagggtgtgagggaccgagcatccagcttggcctgcaggacttcaatcactttctccttctcctgcagctccctgctgagcctgagggccagtggctcaagtccagcttgatctttctcacttttatgatccttggtgctgagtttgctggtgagcctctctgtcagctggcttccctgggcgagttgctcccggaagctctgtcccaggtagtagtcaatgtcattgctccttaggagatcctcaaaagattttactgtatcttttgcatgccgggtgataagataacaaatacctctcccttctcgtattttttgccgtaggtaagacagttcccgggcctgatcctgaatcagggaatcatatttcccaggccacgaggctgatctcagctcctcagccagcttctcttctagtccattttttgggagctgggcctccagctgggatactctctggatgagactctccaggtcctttttggcctgaagccctggagagtagaaagccccagtgccatcagacagccacccctcatcctcatcagggacactatgaggtgaagacccctccaaggtgccaacagctctcagcttccggggtctttccagactagacgaataatcacttgtaactgagagggaccggacccggctcttgaggttttgaatgaccttgttggcattctgcagctgggccttcagatctttgatgtcctttcgtaggaccaagatgttttctgactttccatatacccggaactcttcctgcttccctagctggttctccaagggcttcctctcagaggaactagccagtgttgagccccggcgtccctgctcagagcacagcccctccatcaggaccatttccttgaggctgttgtgctcctcacactcaggactggtggtttcctcccgttcagcctcattctcgcttcggccacaagtctcatagcccaggtcctggaggtccacctggatctgcttgctgtcctgcttcaccaaggattcacctgtaagcataactctgtatttctccagctcgttagcctgagcaaagacagtggcttctgatagcagcagcttctcctggagatcttgatagcgttgtttgcattgtgacagctgggagcgcaggtgctgggtggaccctggtaggctaaacgctgactgaggcccagggtcacgaggctgggactggttatccaattggtgggcatccactgtgaaggtagccccaaggtcaaggctctggggtctggggaaaggcctcacagtcacattcccctcctcttggtgttggtgcttcccaggggaaccaaccagttctgtgtttattctttcaatggtgctggtcagatgcacaaggagctctggagtaagtttactattcccttccttgctactcagcacaagttgttctttgaggaggttgatgatattgtgggcattcttcagttttccctggagctttctgaactcagcctgaaggctactctcactcagaccctctttggttaccacagtctcaaccatcacctcgcccttctccttgtcttcctcgatctcccatccatcagacattgcttctcccatctgctctttcagctccgcattctcaaggcaaaggctcagcatggtgttcctgatgtgggacactgaggagaatcctgcttcctcaatttgagcctttagctccttcagttcctcctcagctttcctcttctcttctaagtgctggtggaactcagccctcaggtggagcatttcttcctgaagacacctgttactgtcccctcccatcggagaaggaggggaaaaagatgggttctgggtctccacagttgccagacttttctccaaagccaccttgacaagttgctggtgactatggtgtgcagcctcctcctcaatactgtcagtgaactcagtgcttgtatcttcggtgtcatcccctgcagctgcacctccaatggcggccagggtctccagcctgtttaagcgctccaagcttcttccaagaacttcttctagccgactgcgtaacacctgagccccttccagttccacctgcagagttcggtctctctcagagctctctggatgggcatggaacttcaccagactgctatagagctgtctctctgcttgtaaggcctcattgagccgactccgttcatctactagtccttctagcatcagcagcaactgttgtcttcggtttcctgaaatttcttgaccctgggattctactgaagcaactttttcccgaagaagtaagacttcctgggtcaggcgttccatagctggtatgtcttcaggatcaaccagttgcatttgcaggtcctttatgagatcttctttaatctgtatgttcctggtcagagactccatatcagcagcctgcacctgcagctcttcttcctgcacagccatcatggactgtagagcagaaagttccatctgactttctctttcttttttagccatgagttcaagttcctctttggcattactcagttctttttccagccctgcaactgtgtccaagtctcctaatgtggatctgggtatgctgacatcctctttggcagtcaatgaagtgctatcatctctggaaggtatctgcattgaaccttgatcagtctgttttccaagacggccagtgggggtaacttcagcttgttggttagagatgggtgcttgggacatcagggagtctctccctcctaaatattggcgcagggcctgtaattctgaatttctttccattaaggcttgcaccaacttctctgcagcagcttggctttcctgctccctggtgctcacagactgaagcaggccttgaatctccatttcatgttccagcacttgtttatttcgatcacttagaaggtcctgcagcatcctttcctttcgctgtagacgctggcacagctcctctgctatctcactctgccctggtccaagtttgcagagcagtgttgcactaagatcctccacttctttgttcctatcatgaagagacgtctgtaactgctgaatgatactctcttgttccttctgccaacggctaaatttggtttccatttcttctttcagccactggaggttttgacaggtagtagataactgttccacttccaggcctttggccctcaggagactctccatactttgcatagtagcttcattggaggagaggacatcgcgcagtctctctaagtcatgatctcgctctctcacagcaagacgaagctggcgcagttctttttctttctcttctagagcagagaatttttcatctatagcccgctccagagcaacagctttatcatgtattcgctggcgaagtttctcaagcaacatttcatttgcttcaagggttttgtctgagttatctcgatactgtaggagctcccgaaattcctgaagcaactgctccttgtgactcagactatggtttaggtgctggatgttttgttcctgggttcgaatctcattgtatttttcagcctcccaggcacgaagctgttggctcttattctgcaattcttcttgtagctgctgcaaggcttttcgcaattcctggttatgtttccaagaagcctctttctgctgttcactctcgtgtgctgcagcctctacaaattgcacacattgtttggcatcagccagttggcgctctttctgtcgtaccaccctctggagcttctgtatttcaagttggctgcagaataaagcactctgaagatcaagcagagctacctgttgctgagctggagaagtaccctctgagctgtgaagttgtccaagctggctttggtgcagcatttctcgaagctttgccattgtgtcattttgaccttcaattacctggtacaactcctcagtctcacgttccctgcttttcagagtttccttgaggttctgaattgtaccatcttgcttttgagacgactcctgagcacactttagttcatagctcatttcattaagtttctcttgaagaatcttgttggtggcctctgtttgctggattttttcctggagttctgccaagtgggaatcagatacagactgctgagttatagtggtctcatgtgaattcagcttttgttgtttcagcaactcttcagtcatgggctgcacttccatgctagttggctcctccaacagatgtagcagttgttgtttctcccgagatagctgttctacaagcctctcctgggcagccaggctctgattcagttcttcaattctcttgtccctctgggccagggcctcagtgtattggtcgggcttgacctggtctcctggtacatcttcccagtttttggtgactcccttcagtttctctgagagctccaggttacactccttctctgcttccaccagagctgccatccgcgcagcttcattctttgctagcctggattcctcctgcagaagctggatcttattctccaagagctcataaacatgctccgtctcctgctgtcgctcctcaaactggcgtcggagctcagcttcattctgactgttgagattctccacatcagcccatgttttatccagatgctgtttcttgtcctggagttctcgtttcaagctctccacttcaaccttcagctcaatgttccgcttgtagatgtcctcccggctggcctcatacttctgttgcatgcgctcctccaggaagtagatgcgcagcttgaggctgaagttctccttcttcaggtcattgaggtgcttctcaaagtctcgaagagcctgggtctgtacctgagggggtttctcaaatgctctcaaggaatatgtctgcacaaacgggaccttttcaccacttctccagatctgtgactgcactggagggcctcgatctttagtgtcactaagaaaagctgctgtgtgactcgttctgggtaccatctccccatcatcctctgcaaaataatctctcgtccaggtctgctccattttccaggctctttccttagtctcaggacgctcctcacccgggaggggaagcagcctgggaaaatgagaagccttgcccacgaatctccagcgcaaaaggcagcagctttttcctccccagctcctttctgcgtcggcggcgaagagagagctctgctccctgcttttttagaaaatggatttgacgtggccgaacctgcggctagccgtgcgacccgcacaagggagggactgttctcagtaggaggctggactcagagcggcgcggcgcccggggctgtttcgtgagctggagccagcggctgcccgggccgcggtgcgcgcactctccaggctgagacacgact

SEQ ID NO: 8832 - RNA, 307 nt, Homo sapiens
  source 1..307: mol_type = other RNA
aagtgtgcagggcactggtgctgctccgaagctcatgaatgcctttgctgcctagcaccatgtgttctgttgattatggccgtttctgagccaggagtagaggaagcagagctggggaggaccagagctggggaattcataccaacatcccggactggaggggacacagctgaatctagggggtaaaggcaaccacagttttcaggagccctggaacacactgcacatgaagcacatgcacacctagccgtccccactgagacctaaggtggcaggactctcctcttacagaattatccatacccca

SEQ ID NO: 8833 - RNA, 1013 nt, Homo sapiens
  source 1..1013: mol_type = other RNA
aagtgtgcagggcactggtgctgctccgaagctcatgaatgcctttgctgcctagcaccatgtgttctgttgattatggccgtttctgagccaggagtagaggaagcagagctggggaggaccagagctggggaattcataccaacatcccggactggaggggacacagctgaatctttcagccccttcttggaattgccataaagtgcctcatagatttgtaactctgactggagggactcaaagagctgctgtttctcttcacactgttgctgcaggagaaccagcttgtgctgcagtctggagtcgttttcctggagggaaaggcgttcctccctgaaatgcaagacctcttgctgcttctccctcaagtcttccaaaagctgctgcctttccaccttctggtgctccagctcctcttccagctcttgaaggtgggatcgagaggacagcagagcctccctcaggctttccatctcctgggagtgctctccagagcaacagctttatcatgtattcgctggcgaagtttctcaagcaacgtttcatttgcttcaagggttttgtctgagttatctcgatactgtaggagctcccgaaattcctgaagcaactgctccttgtgactcagactatggtttaggtgctggacgttttgttcctgggttcgaatctcattgtatttttcagcctcccaggcacgaagctgttggctcttattctgcaattcttgtagctgctgcaaggcttttcgcaattcctgaattaaacatattacatttgatcctccatatctgtaggttctgcatccatggattcaaccaggcctgactccaaaatattttttgaaaacttattattgtgtttgcactgtacatatatggacttttttctttgtcattattccctaaacaataccacataacaactatttacatagcatacgggaggatgtgagtaggttatctgcaaactctacgtcattttgagaggtgacagcgttctggcagtcc

SEQ ID NO: 8834 - RNA, 492 nt, Homo sapiens
  source 1..492: mol_type = other RNA
aagtgtgcagggcactggtgctgctccgaagctcatgaatgcctttgctgcctagcacctctgtgccttgggcttcaaggccagggaagctgcacgctgatctcacaagagacactatctttttgaccagcagcttgccctccgcaatctgctgtcttagggcactgtagtcatcaatgtggccaatgacatggcggccatgcttactggcaaaggagccatcagtagcatcaccctctagcttgggaggggtcttcattactggagaagtatccaaacccaagccatttgttctgttgattatggccgtttctgagccagaagtagaggaagcagagctggggaggaccagagcttgggaattcataccaacatcccggactggaggggacacagcagaatctctctggatgggcatggaacttcaccagactgctatagagctgtctctctgcttgtaaggcctcactgagccgactccgttcatctact

SEQ ID NO: 8835 - RNA, 7143 nt, Homo sapiens
  source 1..7143: mol_type = other RNA
aagtgtgcagggcactggtgctgctccgaagctcatgaatgcctttgctgcctagcacctctgtgccttgggcttcaaggccagggaagctgcacgctgatctcacaagagacactatctttttgaccagcagcttgccctccgcaatctgctgtcttagggcactgtagtcatcaatgtggccaatgacatggcggccatgcttattggcaaaggagccatcagtagcatcaccctctagcttgggaggggtcttcattactggagaagtatccaaacccaagccatttgctctgttgattatgggcgtttctgagccaggagtagaggaagcagagctggggaagaccagagctggggaattcataccaacatcccggactggaggggacacagctgaatcttggaggagcagctgcttgtttccagggtcagtgctggctgggaagttctggttaatggaggaggggctgaggctggctttgccagcaccgctctccagctgctgttgcagctgcagtcgcagacaattgttcccctgaatgctctgctccagctgccctctcagagctcgtacctctgccaccaggtggctcaggtcactgctcaaagggatttggtgacaggcatccaggctgtaagctttcagccccttcttggaattgccataaagtgcctcgtagatttgtagctctgactggagggactcaaagagctgctgtttctcttcacactgttgctgcaggagaaccagcttgtgctgcagtctggagtcgttttcctggagggaaagacgttcctccctgaaatgcaagacctcttgctgcttctccctcaagtcttccaaaagctgctgcctttccaccttctggtgctccagctccttttccagctcttgaaggtgggatcgagaggacagcagagcctccctcaggctttctgtttcctgggagtgctctctggaaacatgactcagttgagcctgaagtcttcgattttcttccctgaggactctgttctcattgcagagctgaggtatggactccaggccctgactgtagaagttagaagtggatccccttccacgagcagtagaggtcagccggtgttccagttgctcccgtaggcagtcattgatgcagatggactcctccaggcgctggcgcaggttccggatttcaccaagatgctcttccagcaggtcagcccctgtgggtttggagttaagctggtacacagaggagcctgaggataggtccccagatacactccctttctgaggcctcatcacatcccacttgccactgctgcccaggtacccaggctctaggattcttcccagttctatggtgccccttggaggagagtgaggctgggcagagttgaggtagtaggaagagtcggcttccaagtcgttgctcagcaatgtagctgtggaagcaggaggaacagtgctggtacctgaatgggcttggttggcctccttgggggtattctggggagttggcaagctgatggggttgctgttggattcggccttagccccctgagatgcactggttgatgatggtttagaagacaacacagcagaatgactcgaatgatggatggaatctgagtgactgggagaagctttcttctcttcatagtgtgtgtactcgctgactatgtccatgtcagagcaggcttccagctcatcagacaggaaagaggtgctgctgggagagcggtgggagtcagacaaggcacggctgctggagggtgtgagggaccgagcatccagcttggcctgcaggacttcaatcactttctccttctcctgcagctccctgctgagcctgagggccagtggctcaagtccagcttgatctttctcacttttatgatccttggtgctgagtttgctggtgagcctctctgtcagctggcttccctgggcgagttgctcccggaagctctgtcccaggtagtagtcaatgtcattgctccttaggagatcctcaaaagattttactgtatcttttgcatgctgggtgataagataacaaatacctctcccttctcgtattttttgccgtaggtaagacagttcccgggcctgatcctgaatcagggaatcatatttcccaggccacgaggctgatctcagctcctcagccagcttctcttctagtccattttctgggagctgggcctccagctgggatactctctggatgagactctccaggtcctttttggcctgaagccctggagagtagaaagccccagtgccatcagacagccacccctcatcctcatcagggacactatgaggtgaagacccctccaaggtgccaacagctctcagcttccggggtctttccagactagacgaataatcacttgtaactgagagggaccggacccggctcttgaggttttgaatgatcttgttggcattctgcagctgggccttcagatcttcgatgtcctttcgtaggaccaagatgttttctgactttccatatacccggaactcttcctgcttccctagctggttctccaagggcttcctctcagaggaactagccagtgttgagccccggcgtccctgctcagagcacagcccctccatcaggaccatttccttgaggctgttgtgctcctcacactcaggactggtggtttcctcccgttcagcctcattctcgcttcggccacaagtctcatagcccaggtcctggaggtccacctggatctgctcgctgtcctgcttcaccaaggattcacctgtaagcataactctgtatttctccagctcgttagcctgagcaaagacagtggcttctgatagcagcagcttctcctggagatcttgatagcgttgtttgcattgtgacagctgggagcgcaggtgctgggtggaccctggtaggctaaacgctgactgaggcccagggtcacgaggctgggactggttatccaactgtgaaaggggccaatacagggatcaggacagtctgaggtcacccccatgcagtgacgaccaccgccccttctgaaccctgtggactttactcaagtctgtcacagcacttctcatgccatttggcagtgacttgctttccagatggagctcctggagcgctgggataatgttttcttcatatctgtatccacagcacacagcacagcaccaatcaggtctacagaggagctctcaggaaatgttttctcagtggtcaaaaagagaccactcatctcccctcacattctgtcccattgattctctcagaatccctgtattctccatttcactgaatcttcagcatggctccttccctaaagaggatcccagtaacccatctgaagaccaggaacagacacctgtgatgagttggtgggcatccactgtgaaggtagccccaaggtcaaggctctggggtctggggaaaggcctcacagtcacattcccctcctcttggtgttggtgcttcccaggggaaccaaccagttctgtgtttattctttcgatggtgctggtcagatgcacaaggagctctggagtaagtttactattcccttccttgctactcagcacaagttgttctttgaggaggttgatgatattgtgggcattcttcagttttccctggagctttctgaactcagcctgaaggctactctcactcagaccctctttggttaccacagtctcaaccatcacctcgcccttctccttgtcttcctcgatctcccatccatcagacattgtttctcccatctgctctttcagctccgcattctcaaggcaaaggctcagcatggtgttcctgatgtgggacactgaggagaatcctgcttcctcaatttgagcctttagctccttcagttcctcctcagctttcctcttctcttctaagtgctggtggatctcagccctcaggtggagcatttcttcctgaagacacctgttactgtcccctcccatcggagaaggaggggaaaaagatgggttctgggtctccacagttgccagacttttctccaaagccaccttgacaagttgctggtgactatggtgtgcagcctcctcctcaatactgtcagtgaactcagtgcttgtatcttcggtgtcatcccctgcagctgcaccttatctccgtaaggaattcgacggagacaaataaatgctcatctcatctcgacactctgccacacaggggttttgtttcttccccttcattctctcttttttaagctagctcacagtcttcttccattatggcagctttaagggttgctcagccttttaccaatttgaattaaaatgctgaaactttttctcccatgtttgaggggtaaagctgactttctctttcttttttagccatgagttcaagttcctctttggcattactcagttctttttccagccctgcaactgtgtccaagtctcctaatgtggatctgggtatgctgacatcctctttggcagtcaatgaagtgctatcatctctggaaggtatctgcattgaaccttgatcagtctgttttccaagacggccagtgggggtaacttcagcttgttggttagagatgggtgcttgggacatcagggagtctctccctcctaaatattggtgcagggcctgtaattctgaatttctttccattaaggcttgcaccaacttctctgcagcagcttggctttcctgctccctggtgctcacagactgaagcaggccttgaatctccatttcatgttccagcacttgtttatttcgatcacttagaaggtcctgcagcatcctttcctttcactgtagacgctggcacagctcctctgctatctcactctgccctggtccaagtttgcagagcaatgttgcactaagatcctccacttctttgttcctatcatgaagagacgtctgtaactgctgaatgatactctcttgttccttctgccaacggctaaatttggtttccatttcttctttcagccactggaggttttgacaggtagtagataactgttccacttccaggcctttggccctcaggagactctccatagtttgcatagtagcttcattggaggagaggacatcgcgcagtctctctaggtcatgatctcgctctctcacagcaagacgaagctggcgcagttctttttctttctcttctagagcagagaatttttcatctatagcccgctccagagcaacagctttatcacgtattcgctggcgaagtttctcaagcaacatttcatttgcttcaagggttttgtctgagttatctcgatactgtaggagctcccgaaattcctgaagcaactgctccttgtgactcagactatggtttaggtgctggatgttttgttcctgggttcgaatctcattgtatttttcagcctcccaggcacgaagctgttggctcttattctgcaatacttcttgtagctgctgcaaggcttttcgcaattcctggttatgtttccaagaagcctctttctgctgttcactctcgtgtgctgcagcctctacaaattgcacacattgtttggcatcagccagttggcgctctttctgtcgtaccaccctctggagcttctgtatttcaagttggctgcagaataaagcactctgaagatcaagcagagctacctgttgctgagctggagaagtaccctctgagctgtgaagttgtccaagctggctttggtgcagcatttctcgaagctttgccattgtgtcattttgaccttcaattacctggtacaactcctcagtctcacgttccctgcttttcagagtttccttgaggttctgaattgtaccatcttgcttttgagacaactcctgagcacactttagttcatagctcatttcattaagtttctcttgaagaatcttgttggtggcctctgtttgctggattttttcctggagttctgccaagtgggaatcagatacagactgctgagttatagtggtctcatgtgaattcagcttttgttgtttcagcaactcttcagtcatgggctgcacttccatgctagttggctcctccaacagatgtagcagttgttgtttctcccgagatagctgttctacaagcctctcctgggcagccaggctctgattcagttcttcaattctcttgtccctctgggccagggtctcagtgtattggtcgggcttgacctggtctcctggtacatcttcccagtttttggtgactcccttcagtttctctgagagctccaggttacactccttctctgcttccaccagagctgccatccgcgcagcttcattctttgctagcctggattcctcctgcagaagctggatcttattctccaagagctcataaacatgctccgtctcctgctgtcgctcctcaaactggcgtcggagctcagcttcattctgactgttgagattctccacatcacccccgcttgtagatgtcctcccggctggcctcatacttctgttgcatgcgctcctccaggaagtagatgagcagcttgaggctgaagttctccttcttcaggtcattgaggtgcttctcaaagtctcgaagagcctgggtctgtacctgagggggtttctcaaatgctctcaaggaatatgtctgcacaaacgggaccttttcaccacttctccagatctgtgactgcactggagggcctcgatctttagtgtcactaagaaaagctgctgtgtgactcgttctgggtaccatctccccatcatcctctgcaaaataatctctcgtccaggtctgctccattttccaggctctttccttagtctcaggacgctcctcacccgggaggggaagcagcctgggaaaatgagaagccttgcccacgaatctccagcgcaaaaggcagcagctttttcctccccagctcctttctgcgtcggcggcgaagagagagctctgctccctgcttttttagaaaatggatttgacgtggccgaacctgcggctagccgtgagacccgcacgagggagggactgttctcagtaggaggctggactcggagcggcgcggcgcccggggctgtttcgtgagctggagccagcggctgcccgggcggcggtgcgcgcactctccaggctgagacacgactggctggc

SEQ ID NO: 8836 - RNA, 7010 nt, Homo sapiens
  source 1..7010: mol_type = other RNA
aagtgtgcagggcactggtgctgctccgaagctcatgaatgcctttgctgcctagcacctctgtgccttgggcttcaaggccagggaagctgcacgctgatctcacaagagacactatctttttgaccagcagcttgccctccgcaatctgctgtcttagggcactgtagtcatcaatgtggccaatgacatggcggccatgcttattggcaaaggagccatcagtagcatcaccctctagcttgggaggggtcttcattactggagaagtatccaaacccaagccatttgctctgttgattatgggcgtttctgagccaggagtagaggaagcagagctggggaagaccagagctggggaattcataccaacatcccggactggaggggacacagctgaatcttggaggagcagctgcttgtttccagggtcagtgctggctgggaagttctggttaatggaggaggggctgaggctggctttgccagcaccgctctccagctgctgttgcagctgcagtcgcagacaattgttcccctgaatgctctgctccagctgccctctcagagctcgtacctctgccaccaggtggctcaggtcactgctcaaagggatttggtgacaggcatccaggctgtaagctttcagccccttcttggaattgccataaagtgcctcgtagatttgtagctctgactggagggactcaaagagctgctgtttctcttcacactgttgctgcaggagaaccagcttgtgctgcagtctggagtcgttttcctggagggaaagacgttcctccctgaaatgcaagacctcttgctgcttctccctcaagtcttccaaaagctgctgcctttccaccttctggtgctccagctccttttccagctcttgaaggtgggatcgagaggacagcagagcctccctcaggctttctgtttcctgggagtgctctctggaaacatgactcagttgagcctgaagtcttcgattttcttccctgaggactctgttctcattgcagagctgaggtatggactccaggccctgactgtagaagttagaagtggatccccttccacgagcagtagaggtcagccggtgttccagttgctcccgtaggcagtcattgatgcagatggactcctccaggcgctggcgcaggttccggatttcaccaagatgctcttccagcaggtcagcccctgtgggtttggagttaagctggtacacagaggagcctgaggataggtccccagatacactccctttctgaggcctcatcacatcccacttgccactgctgcccaggtacccaggctctaggattcttcccagttctatggtgccccttggaggagagtgaggctgggcagagttgaggtagtaggaagagtcggcttccaagtcgttgctcagcaatgtagctgtggaagcaggaggaacagtgctggtactttctcccaactgcttctgcagcatctgtagctcctgctgagactcagccaaggagacctctggtgtctcacagcagccaaggaggggagggccagtggggctgaaaggcaggaagctggatggagctgagggcaatggtgcctgaggaaggctagccagcttgggtatggagtgaaaatgaaagcctgaatgggcttggttggcctccttgggggtattctggggagttggcaagctgatggggttgctgttggattcggccttagccccctgagatgcactggttgatgatggtttagaagacaacacagcagaatgactcgaatgatggatggaatctgagtgactgggagaagctttcttctcttcatagtgtgtgtactcgctgactatgtccatgtcagagcaggcttccagctcatcagacaggaaagaggtgctgctgggagagcggtgggagtcagacaaggcacggctgctggagggtgtgagggaccgagcatccagcttggcctgcaggacttcaatcactttctccttctcctgcagctccctgctgagcctgagggccagtggctcaagtccagcttgatctttctcacttttatgatccttggtgctgagtttgctggtgagcctctctgtcagctggcttccctgggcgagttgctcccggaagctctgtcccaggtagtagtcaatgtcattgctccttaggagatcctcaaaagattttactgtatcttttgcatgctgggtgataagataacaaatacctctcccttctcgtattttttgccgtaggtaagacagttcccgggcctgatcctgaatcagggaatcatatttcccaggccacgaggctgatctcagctcctcagccagcttctcttctagtccattttctgggagctgggcctccagctgggatactctctggatgagactctccaggtcctttttggcctgaagccctggagagtagaaagccccagtgccatcagacagccacccctcatcctcatcagggacactatgaggtgaagacccctccaaggtgccaacagctctcagcttccggggtctttccagactagacgaataatcacttgtaactgagagggaccggacccggctcttgaggttttgaatgatcttgttggcattctgcagctgggccttcagatcttcgatgtcctttcgtaggaccaagatgttttctgactttccatatacccggaactcttcctgcttccctagctggttctccaagggcttcctctcagaggaactagccagtgttgagccccggcgtccctgctcagagcacagcccctccatcaggaccatttccttgaggctgttgtgctcctcacactcaggactggtggtttcctcccgttcagcctcattctcgcttcggccacaagtctcatagcccaggtcctggaggtccacctggatctgctcgctgtcctgcttcaccaaggattcacctgtaagcataactctgtatttctccagctcgttagcctgagcaaagacagtggcttctgatagcagcagcttctcctggagatcttgatagcgttgtttgcattgtgacagctgggagcgcaggtgctgggtggaccctggtaggctaaacgctgactgaggcccagggtcacgaggctgggactggttatccaattggtgggcatccactgtgaaggtagccccaaggtcaaggctctggggtctggggaaaggcctcacagtcacattcccctcctcttggtgttggtgcttcccaggggaaccaaccagttctgtgtttattctttcgatggtgctggtcagatgcacaaggagctctggagtaagtttactattcccttccttgctactcagcacaagttgttctttgaggaggttgatgatattgtgggcattcttcagttttccctggagctttctgaactcagcctgaaggctactctcactcagaccctctttggttaccacagtctcaaccatcacctcgcccttctccttgtcttcctcgatctcccatccatcagacattgtttctcccatctgctctttcagctccgcattctcaaggcaaaggctcagcatggtgttcctgatgtgggacactgaggagaatcctgcttcctcaatttgagcctttagctccttcagttcctcctcagctttcctcttctcttctaagtgctggtggatctcagccctcaggtggagcatttcttcctgaagacacctgttactgtcccctcccatcggagaaggaggggaaaaagatgggttctgggtctccacagttgccagacttttctccaaagccaccttgacaagttgctggtgactatggtgtgcagcctcctcctcaatactgtcagtgaactcagtgcttgtatcttcggtgtcatcccctgcagctgcaccttatctccgtaaggaattcgacggagacaaataaatgctcatctcatctcgacactctgccacacaggggttttgtttcttccccttcattctctcttttttaagctagctcacagtcttcttccattatggcagctttaagggttgctcagccttttaccaatttgaattaaaatgctgaaactttttctcccatgtttgaggggtaaagctgactttctctttcttttttagccatgagttcaagttcctctttggcattactcagttctttttccagccctgcaactgtgtccaagtctcctaatgtggatctgggtatgctgacatcctctttggcagtcaatgaagtgctatcatctctggaaggtatctgcattgaaccttgatcagtctgttttccaagacggccagtgggggtaacttcagcttgttggttagagatgggtgcttgggacatcagggagtctctccctcctaaatattggtgcagggcctgtaattctgaatttctttccattaaggcttgcaccaacttctctgcagcagcttggctttcctgctccctggtgctcacagactgaagcaggccttgaatctccatttcatgttccagcacttgtttatttcgatcacttagaaggtcctgcagcatcctttcctttcactgtagacgctggcacagctcctctgctatctcactctgccctggtccaagtttgcagagcaatgttgcactaagatcctccacttctttgttcctatcatgaagagacgtctgtaactgctgaatgatactctcttgttccttctgccaacggctaaatttggtttccatttcttctttcagccactggaggttttgacaggtagtagataactgttccacttccaggcctttggccctcaggagactctccatagtttgcatagtagcttcattggaggagaggacatcgcgcagtctctctaggtcatgatctcgctctctcacagcaagacgaagctggcgcagttctttttctttctcttctagagcagagaatttttcatctatagcccgctccagagcaacagctttatcacgtattcgctggcgaagtttctcaagcaacatttcatttgcttcaagggttttgtctgagttatctcgatactgtaggagctcccgaaattcctgaagcaactgctccttgtgactcagactatggtttaggtgctggatgttttgttcctgggttcgaatctcattgtatttttcagcctcccaggcacgaagctgttggctcttattctgcaatacttcttgtagctgctgcaaggcttttcgcaattcctggttatgtttccaagaagcctctttctgctgttcactctcgtgtgctgcagcctctacaaattgcacacattgtttggcatcagccagttggcgctctttctgtcgtaccaccctctggagcttctgtatttcaagttggctgcagaataaagcactctgaagatcaagcagagctacctgttgctgagctggagaagtaccctctgagctgtgaagttgtccaagctggctttggtgcagcatttctcgaagctttgccattgtgtcattttgaccttcaattacctggtacaactcctcagtctcacgttccctgcttttcagagtttccttgaggttctgaattgtaccatcttgcttttgagacaactcctgagcacactttagttcatagctcatttcattaagtttctcttgaagaatcttgttggtggcctctgtttgctggattttttcctggagttctgccaagtgggaatcagatacagactgctgagttatagtggtctcatgtgaattcagcttttgttgtttcagcaactcttcagtcatgggctgcacttccatgctagttggctcctccaacagatgtagcagttgttgtttctcccgagatagctgttctacaagcctctcctgggcagccaggctctgattcagttcttcaattctcttgtccctctgggccagggtctcagtgtattggtcgggcttgacctggtctcctggtacatcttcccagtttttggtgactcccttcagtttctctgagagctccaggttacactccttctctgcttccaccagagctgccatccgcgcagcttcattctttgctagcctggattcctcctgcagaagctggatcttattctccaagagctcataaacatgctccgtctcctgctgtcgctcctcaaactggcgtcggagctcagcttcattctgactgttgagattctccacatcacccccgcttgtagatgtcctcccggctggcctcatacttctgttgcatgcgctcctccaggaagtagatgagcagcttgaggctgaagttctccttcttcaggtcattgaggtgcttctcaaagtctcgaagagcctgggtctgtacctgagggggtttctcaaatgctctcaaggaatatgtctgcacaaacgggaccttttcaccacttctccagatctgtgactgcactggagggcctcgatctttagtgtcactaagaaaagcagaaggagcccaagaaaaagcacccagatgcttcagtcaacttcttagaattcttcttttttttatgttcagaaaagatggaaattcatttctgctgtgtgactcgttctgggtaccatctccccatcatcctctgcaaaataatctctcgtccaggtctgctccattttccaggctctttccttagtctcaggacgctcctcacccgggaggggaagcagcctgggaaaatgagaagccttgcccacgaatctccagcgcaaaaggcagcagctttttcctccccagctcctttctgcgtcggcggcgaagagagagctctgctccctgcttttttagaaaatggatttgacgtggccgaacctgcggctagccgtgagacccgcacgagggagggactgttctcagtaggaggctggactcggagcggcgcggcgcccggggctgtttcgtgagctggagccagcggctgcccgggcggcggtgcgcgcactctccaggctgagacacgactggctggc

SEQ ID NO: 8837 - RNA, 70 nt, Homo sapiens
  source 1..70: mol_type = other RNA
aagttggctgcagttaaggtggcaccatcagctgattagccaccttaactgcagccaactttcattcccc

SEQ ID NO: 8838 - RNA, 167 nt, Homo sapiens
  source 1..167: mol_type = other RNA
aataatatcacagtaggtgtatgaaatacttgcatcggatgagttgcagacccaatactgcttctgagcttcagtaaatatggaagaaaacagggtggaaaaaaacagaaatggtaacatgattcaatatctccaaagctttacaaatgcaaagaggatcagtaact

SEQ ID NO: 8839 - RNA, 171 nt, Homo sapiens
  source 1..171: mol_type = other RNA
aataatatcacagtaggtgtatgaaatacttgcatcggatgagttgcagacccaatactgcttctgagcttcagtaaatatggaagaaaacagggtggaaaaaaacagaaatggtaacatgattcaatatctccaaagctttacaaatgcaaagaggatcagtaactaatc

SEQ ID NO: 8840 - RNA, 2705 nt, Homo sapiens
  source 1..2705: mol_type = other RNA
aatagctcagaatgtcagttctgtttgttaatggcaagattccaattttagaattttgacctcgtctgtactcctttatacctaattttaaagaaatatgccattattatctggccccagactacatattttttaaatttaagtttttattgatgtatttcttgcaatatacttgggaaggatgccaaaatgttaacattgacatcaataaaaaataatataaatgctttaaatgaaagagtgaaagaaaagaagaaagataaaccatttcatgtctgtagccatattattgtcatcattaaagtagagatacagtaaaagtaagaagagataaaagaatggcacacacatgtatccaatcatatttatctcaaaaatatgccaaatttccatttaaaatgtcatggcatttattatttttaaaccattcaaaatttcttcttactgaggttcttgaagtgggctcctataatttgagtagttgaagacattatttgcctaatatgaagttttcagttattagtgtagttagaatgtaatttctcttaatttgcactaaaacttataaagtttgatacttttttgcaacctaaaactaggctttatgtttattgtgatgtttgggatccttaaataatttcttattactaaaatatctttatacattgggaatcatttaaatatgtattaggctaaaattggtactatgaaatcagtgtcatactttttacaggacacattataactgaatagagtttcaaagaaaggagtaaatagttattagaactttactgcatattcctgccaataatattgcaaagaaatgttcttgtgggaattgaacaagatggacttttctgttcagctactcccccattccaatttctgaaaaaaaaaacaaaaaagatgttccttaattatattaacctttcatctgagacagggtgtggtggcccacacctgtaatcccagcactttgggaagctgaggcgagcagatcacttgaggtcaggagtttgagaccagcctggccaacatggtgaaaccctttctctactaaaaatacaaaaattcaccaggcctggtggtgtgctgtggtcccagctactcgggaggctgaggcaggagaatcgcttgaacccgggaggtagaggttgcagtgagccaagatggcaccactacactctggcctgggcaacagagcaagactccatctaaaaaaaaaacaaaaaaaaaaaattttcatctgagagcaggtaaaccattgcaaagtcatgccccaatcgttgtacaatatccatttcctacagttgacataacaaattccaaaaaacaggtcacctaaaacaacagaaatttactctctcacagtttcggggctaaaagtctgaaatcaaggtaccatcagtgctgtgtttttgctgacagctttggggagaatcctttcttgcctcttctagcttctggtgatacttgccagcaatccttggtatgtgtgttggtttgtagatgctccactccaaccacgtggtcaccttctctctgtgtgtcttcaggtagtcttcctctgtgcccctctcatgtccacatttctcccttcacttctggattgcgaggagtataggtcatattaaggcttaatgttccaattctatttttaaattatccgtttataaattaagccactttaagcctgatgctcatcctcgtagttctctttacagctctctctcctctttaagtaatcagtttcttctctttctcttttatgtcaaaagccttcctgagataatgaaggtcaattctttctccgttagggatatctcaaatctctccaagggcttcttcaaatctctccgagggcttcatttcctatgcagagtgtgctatccttaatcacttgaagaatcttttgacagagccttttgtaacgtttttgtagtttcctgctttacagaatttgcaggcttagtaaaagcatggatagaaccagagccactgcaagcagagccaaaggtggaaggatagtgaggcagatccttgacctcaatgctccctaaaaattataaacagcattctctttcattcctggtaagtttccacttccttttgcattttctcataaagaaatccatgtatccttacagtaaattttcttgtttagctttagctagtcatctagatttctggtttttgcagccaaacaacccctaagagatctatgtcttagtggggccaatttcaatcccatttaattcaattcaaccgatgtttattgaatacctattgtgtctcttatacccaataattggggttgagtcttgaatctggcctatgactggaatctatgaaagattcaaagggaaaaataggcataggttatgatgagctataaaaaaagaaacgagacagaacataatgtagagttcttagctctccccacccagatttatgttctgagttttctttaacattctgtccaatcgagtgcgagtgggctgagacgtgggtggcagagctgagacacggcccctctaactgtctcatgtacaaacttgaggggtaagaggaagtttgacacaggaaataacagccagcagccgggctctctgacgaacactacccagtgaagccttttaattaggcaagatcatttttgttaaatctgctcagaaaatactgccttaatctctgaagataataaa

SEQ ID NO: 8841 - RNA, 30 nt, Homo sapiens
  source 1..30: mol_type = other RNA
aataggccacggatctgggcaaaatgtcct

SEQ ID NO: 8842 - RNA, 284 nt, Homo sapiens
  source 1..284: mol_type = other RNA
aatcactaaccacacggccagggcaggctttgagtgccaggctgaggggtttgggactcttcctttacagaagatcaagtgtccccccttctcccacctcccaatccttccctccaataaagtctccggtttttggttccagttcctggtttctgtccctcacggtgcccagatgtactccctttttatgtctaagctagattgcaagggcttccacaacacttaccagacagctgaggtcatgaggcttagtgctaatgaggagacaggagaaatgagacaag

SEQ ID NO: 8843 - RNA, 447 nt, Homo sapiens
  source 1..447: mol_type = other RNA
aatcctttgtccctgggtgagagccatgcctgacttgtctttctttcctcttcctcttcttcaagggttcttcctgaggtcaggagttcgagatcagcctgggcaacacggtgaaaccccgtctctactaaaaatacaaaattagccgggcgtggtggcacatgcctgtaatcccagctactcgggaggctgaggcaggagaatcgcttgaacctgggaggcggaggatgcggtgagccgaaatcgcgccattgcactccagcctggacaacaagagtaaatctccgtctcaccaaaaaaaaaaaaaaagaaaaaaaaaaaggtctgtagcgagcccgggaactggctgcggaaacggggcacggcggttcgcaagtttaatccatactgagggacactcacgctcggcggcgtcacccgcacccaacacgatccgcttccggaact

SEQ ID NO: 8844 - RNA, 118 nt, Homo sapiens
  source 1..118: mol_type = other RNA
aatcctttgtccctgggtgagagccatgcctgacttgtctttctttcctcttcctcttcttcaagggttcttcgctcggcggcgtcacccgcacccaacacgatccgcttccggaact

SEQ ID NO: 8845 - RNA, 1753 nt, Homo sapiens
  source 1..1753: mol_type = other RNA
aatcctttgtccctgggtgagagcctgcagcctttctggaggtaatgtgagagccgccccacagaggccaggaggaggccaaagtatggtggggagggcttgataggcctggacaggaactcagggtggtactgaaccccaacaaaaaagggatgatcttctaactccacaatttccattctctctccttcaacatcttggccaacaaacttcaagccttgttcttccaaacactttttccagactggattcacctcaaatcggtggcggtgcctctcttccaagtagtctgcgtctccatagagtttcccacgggatgactggtcgtagggtcaaactctgtagaattggcatcttgccatcccagcacgtttcttgagaattcaaccactgccaactgcatccctaagcacacgcccaaaaaaggctttttctgattccgagcccaggcaattgcttggatttttccttctgttcctcgaacaccaaatcctcctggaaccagcactccatgagcactacagagcttctgccaagcttcgtggtagcgcacgggctcttcttgcgaggtgatgggctccaagtccgcagaatctatgtacttgatttccaatttgtggttgatggccagtgcagaatgctccagagccttaatgacagaggcataggagtctgagaacttcgtgtatttgcccacaagggcaatagagcaggtctccagcaagcgatcatatctgtcagccatctctttccatttcatcagcatttttcttggctgcctctcaataggaaggtcaagtcttcgaagaaaataatctacaaccccttgctcctctaacaacaaggggactcggtagatggatgagacatcgtggacacagatcacttgttcaggctcaacatggcagaacattgatattttctccttcactgatgtgtcaagtggatttgagcacctgcatacaaccagatctggggaaagcccaagtcctctaagttcccgaacactattctgggtaggtttagtcttctgttcccctgttgaacttggctggggaactagactgacgtggatgttacaaaagttctctcttttgaccttgaattggaactgacggaaggcctcaataaagggcatgctttctatgtcccccacggttccaccaagctcaataacacacacttgaggttccaggccatcttcatctacaggtattaacgcctgtctcatcacccactcctggattgcatctgtgatatgagggacaacttggacagttttccccaagtaatctcctttccgttccttgttaatgacatactggtatatctttccagtggtcagattattgtccttggtgaggcggatgtcaaggaaccgctcatagttacccaggtcaaggtctacttccccaccatcatccagcacaaaaacctcaccatgctcataaggagagaatgttcctgcatcaatgttaatgtaggggtcaattttgattgaagttacatgtaaaccacatgacttgagtattgtgcccacactgctggcaatgattccttttccaattcctgatataacaccaccagtaaccagaatgtacttcattttactctttgacctgcggccggcttcagatcctcccgtcagcgacagagctgggccggcgacgcgcgcggagccccggacagccagtgaacaaccccgaccgcatgcgcccggcagtctttcacggaggcgggctctaggctgtgc

SEQ ID NO: 8846 - RNA, 1751 nt, Homo sapiens
  source 1..1751: mol_type = other RNA
aatcctttgtccctgggtgagagcctgcagcctttctggaggtaatgtgagagccgccccacagaggccaggaggaggccaaagtatggtggggagggcttgataggcctggacaggaactcagggtggtactgaaccccaacaaaaaagggatgatcttctaactccacaatttccattctctctccttcaacatcttggccaacaaacttcaagccttgttcttccaaacactttttccagactggattcacctcaaatcggtggcggtgcctctcttccaagtagtctgcgtctccatagagtttcccacgggatgactggtcgtagggtcaaactctgtagaattggcatcttgccatcccagcacgtttcttgagaattcaaccactgccaactgcatccctaagcacacgcccaaaaaaggctttttctgattccgagcccaggcaattgcttggatttttccttctgttcctcgaacaccaaatcctcctggaaccagcactccatgagcactacagagcttctgccaagcttcgtggtagcgcacgggctcttcttgcgaggtgatgggctccaagtccgcagaatctatgtacttgatttccaatttgtggttgatggccagtgcagaatgctccagagccttaatgacagaggcataggagtctgagaacttcgtgtatttgcccacaagggcaatagagcaggtctccagcaagcgatcatatctgtcagccatctctttccatttcatcagcatttttcttggctgcctctcaataggaaggtcaagtcttcgaagaaaataatctacaaccccttgctcctctaacaacaaggggactcggtagatggatgagacatcgtggacacagatcacttgttcaggctcaacatggcagaacattgatattttctccttcactgatgtgtcaagtggatttgagcacctgcatacaaccagatctggggaaagcccaagtcctctaagttcccgaacactattctgggtaggtttagtcttctgttcccctgttgaacttggctggggaactagactgacgtggatgttacaaaagttctctcttttgaccttgaattggaactgacggaaggcctcaataaagggcatgctttctatgtcccccacggttccaccaagctcaataacacacacttgaggttccaggccatcttcatctacaggtattaacgcctgtctcatcacccactcctggattgcatctgtgatatgagggacaacttggacagttttccccaagtaatctcctttccgttccttgttaatgacatactggtatatctttccagtggtcagattattgtccttggtgaggcggatgtcaaggaaccgctcatagttacccaggtcaaggtctacttccccaccatcatccagcacaaaaacctcaccatgctcataaggagagaatgttcctgcatcaatgttaatgtaggggtcaattttgattgaagttacatgtaaaccacatgacttgagtattgtgcccacactgctggcaatgattccttttccaattcctgatataacaccaccagtaaccagaatgtacttcattttactctttgactttggcatggtcaggacattttcctcctcaggaacgttccatgtgaagccaaattatgataaaaataaactaaggaacaagaaaactaaggagttgtgctcgaagcattcccccgccccaccccctccccag

SEQ ID NO: 8847 - RNA, 3049 nt, Homo sapiens
  source 1..3049: mol_type = other RNA
aatcctttgtccctgggtgagagcctgcagcctttctggaggtaatgtgagagccgccccacagaggccaggaggaggccaaagtatggtggggagggcttgataggcctggacaggaactcagggtggtactgaaccccaacaaaaaagggatgatcttctaactccacaatttccattctctctccttcaacatcttggccaacaaacttcaagccttgttcttccaaacactttttccagactggattcacctcaaatcggtggcggtgcctctcttccaagtagtctgcgtctccatagagtttcctcatgactgagttcttggtctggaacagggttctcctcttgcccagcctcatggttccgcccatctgccctgggttgtgttctggcatgtctacgaccacgggatgactggtcgtagggtcaaactctgtagaattggcatcttgccatcccagcacgtttcttgagaattcaaccactgccaactgcatccctaagcacacgcccaaaaaaggctttttctgattccgagcccaggcaattgcttggatttttccttctgttcctcgaacaccaaatcctcctggaaccagcactccatgagcactacagagcttctgccaagcttcgtggtagcgcacgggctcttcttgcgaggtgatgggctccaagtccgcagaatctatgtactggatgttattcagacaggggagaaaagcaggctcgtgaccccaggctgtgcgttcttaatttttaaataatattatcattttatcaaagttgtctttcttgattctggctttaaagtgatcatcttaatactggctttaaagtgatcaacttaatatatttaataacttaaacattttttaaatatgaggttttaaaatacaacagtttccttcaaaatcattaaattcccaaatctctctctttctgcactctactgtgttcaggatcgggtctcagctaagcctctgcagcagactctagagggctttctgttcaatgacagcctcctcagcccatcttccgcccagcttttgtgggttttttctttttctttctaccatattgaagcataattcacatacaataaaatacaagcattttaagtgcatactttgaagagttttgtcaaacatacacaccaagatatagaatgagccgggcgtggtggctcacacctataatcccagcactttggaaggccgaggcgggtggatcacttgaggtcaggagttcgagactagcctggcaaacatggtgaaaccccatctctactaaaaatacaaaaaaaaaaaaaaaatagctgggtgtggtggcatgcacctgtagtcccagctacccaagaggctgaggcaggagaactgcttgaacctggaaggcagaggttgcagtgaactgggatcatgccactgcactccagcctgggtgacagagcgagactccatctcaaacaaaacaaaacaaaacaaaacaaaacaaaacaaaacaaaacataagttaccatcttcccagaatgtgcccctctacctcctaccccaaacaacctcagatccaatttctatcatcacagattcgttttgcctcttatagaacatcatataaatggagccaaatagtatataaccttttgtgtctggcttcttttgcttagtgtttttgaagttcatccatgttgctgtgtttatcagttgtttgttccttttcttttttaacttttttttgcagagacgggggtctcgctatgttgaccaggctgctctcgaactactggtcttaggcgatcctcccacagcagagcctccctaagtgttgggattatgggcttgagccagtcagtgttcagcctggtttcttccttttcattgctgagtggtttctacttgatttccaatttgtggttgatggccagtgcagaatgctccagagccttaatgacagaggcataggagtctgagaacttcgtgtatttgcccacaagggcaatagagcaggtctccagcaagcgatcatatctgtcagccatctctttccatttcatcagcatttttcttggctgcctctcaataggaaggtcaagtcttcgaagaaaataatctacaaccccttgctcctctaacaacaaggggactcggtagatggatgagacatcgtggacacagatcacttgttcaggctcaacatggcagaacattgatattttctccttcactgatgtgtcaagtggatttgagcacctgcatacaaccagatctggggaaagcccaagtcctctaagttcccgaacactattctgggtaggtttagtcttctgttcccctgttgaacttggctggggaactagactgacgtggatgttacaaaagttctctcttttgaccttgaattggaactgacggaaggcctcaataaagggcatgctttctatgtcccccacggttccaccaagctcaataacacacacttgaggttccaggccatcttcatctacaggtattaacgcctgtctcatcacccactcctggattgcatctgtgatatgagggacaacttggacagttttccccaagtaatctcctttccgttccttgttaatgacatactggtatatctttccagtggtcagattattgtccttggtgaggcggatgtcaaggaaccgctcatagttacccaggtcaaggtctacttccccaccatcatccagcacaaaaacctcaccatgctcataaggagagaatgttcctgcatcaatgttaatgtaggggtcaattttgattgaagttacatgtaaaccacatgacttgagtattgtgcccacactgctggcaatgattccttttccaattcctgatataacaccaccagtaaccagaatgtacttcattttactctttgacctgcggccggcttcagatcctcccgtcagcgacagagctgggccggcgacgcgcgcggagccccggacagccagtgaacaaccccgaccgcatgcgcccggcagtctttcacggaggcgggctctaggctgtgc

SEQ ID NO: 8848 - RNA, 1340 nt, Homo sapiens
  source 1..1340: mol_type = other RNA
aatcctttgtccctgggtgagagcctgcagcctttctggaggtaatgtgagagccgccccacagaggccaggaggaggccaaagtatggtggggagggcttgataggcctggacaggaactcagggtggtactgaaccccaacaaaaaagggatgatcttctaactccacaatttccattctctctccttcaacatcttggccaacaaacttcaagccttgttcttccaaacactttttccagactggattcacctcaaatcggtggcggtgcctctcttccaagtagtctgcgtctccatagagtttcctcatgactgagttcttggtctggaacagggttctcctcttgcccagcctcatggttccgcccatctgccctgggttgtgttctggcatgtctacgaccacgggatgactggtcgtagggtcaaactctgtagaattggcatcttgccatcccagcacgtttcttgagaattcaaccactgccaactgcatccctaagcacacgcccaaaaaaggctttttctgattccgagcccaggcaattgcttggatttttccttctgttcctcgaacaccaaatcctcctggaaccagcactccatgagcactacagagcttctgccaagcttcgtggtagcgcacgggctcttcttgcgaggtgatgggctccaagtccgcagaatctatgtacttgatttccaatttgtggttgatggccagtgcagaatgctccagagccttaatgacagaggcataggagtctgagaacttcgtgtatttgcccacaagggcaatagagcaggtctccagcaagcgatcatatctgtcagccatctctttccatttcatcagcatttttcttggctgcctctcaataggaaggtcaagtcttcgaagaaaataatctacaaccccttgctcctctaacaacaaggggactcggtagatggatgagacatcgtggacacagatcacttgttcaggctcaacatggcagaacattgatattttctccttcactgatgtgtcaagtggatttgagcacctgcatacaaccagatctggggaaagcccaagtcctctaagttcccgaacactattctgggtaggtttagtcttctgttcccctgttgaacttggctggggaactagactgacgtggatgttacaaaagttctctcttttgaccttgaattggaactgacggaaggcctcaataaagggcatgctttctatgtcccccacggttccaccaagctagaagaacaaagttgtttcagaggttaggcactaaacccttctctggcagtttagttttctaacaactgttct

SEQ ID NO: 8849 - RNA, 1788 nt, Homo sapiens
  source 1..1788: mol_type = other RNA
aatcctttgtccctgggtgagagcctgcagcctttctggaggtaatgtgagagccgccccacagaggccaggaggaggccaaagtatggtggggagggcttgataggcctggacaggaactcagggtggtactgaaccccaacaaaaaagggatgatcttctaactccacaatttccattctctctccttcaacatcttggccaacaaacttcaagccttgttcttccaaacactttttccagactggattcacctcaaatcggtggcggtgcctctcttccaagtagtctgcgtctccatagagtttcctcatgactgagttcttggtctggaacagggttctcctcttgcccagcctcatggttccgcccatctgccctgggttgtgttctggcatgtctacgaccacgggatgactggtcgtagggtcaaactctgtagaattggcatcttgccatcccagcacgtttcttgagaattcaaccactgccaactgcatccctaagcacacgcccaaaaaaggctttttctgattccgagcccaggcaattgcttggatttttccttctgttcctcgaacaccaaatcctcctggaaccagcactccatgagcactacagagcttctgccaagcttcgtggtagcgcacgggctcttcttgcgaggtgatgggctccaagtccgcagaatctatgtacttgatttccaatttgtggttgatggccagtgcagaatgctccagagccttaatgacagaggcataggagtctgagaacttcgtgtatttgcccacaagggcaatagagcaggtctccagcaagcgatcatatctgtcagccatctctttccatttcatcagcatttttcttggctgcctctcaataggaaggtcaagtcttcgaagaaaataatctacaaccccttgctcctctaacaacaaggggactcggtagatggatgagacatcgtggacacagatcacttgttcaggctcaacatggcagaacattgatattttctccttcactgatgtgtcaagtggatttgagcacctgcatacaaccagatctggggaaagcccaagtcctctaagttcccgaacactattctgggtaggtttagtcttctgttcccctgttgaacttggctggggaactagactgacgtggatgttacaaaagttctctcttttgaccttgaattggaactgacggaaggcctcaataaagggcatgctttctatgtcccccacggttccaccaagctcaataacacacacttgaggttccaggccatcttcatctacaggtattaacgcctgtctcatcacccactcctggattgcatctgtgatatgagggacaacttggacagttttccccaagtaatctcctttccgttccttgttaatgacatactggtatatctttccagtggtcagattattgtccttggtgaggcggatgtcaaggaaccgctcatagttacccaggtcaaggtctacttccccaccatcatccagcacaaaaacctcaccatgctcataaggagagaatgttcctgcatcaatgttaatgtaggggtcaattttgattgaagttacatgtaaaccacatgacttgagtattgtgcccacactgctggcaatgattccttttccaattcctgatataacaccaccagtaaccagaatgtacttcattttactctttgaccacggaggatttatcactggtccccagcttcagaggtccaggatcgtccatttggtcagcaaacccaaatgt

SEQ ID NO: 8850 - RNA, 2241 nt, Homo sapiens
  source 1..2241: mol_type = other RNA
aatcctttgtccctgggtgagagcctgcagcctttctggaggtaatgtgagagccgccccacagaggccaggaggaggccaaagtatggtggggagggcttgataggcctggacaggaactcagggtggtactgaaccccaacaaaaaagggatgatcttctaactccacaatttccattctctctccttcaacatcttggccaacaaacttcaagccttgttcttccaaacactttttccagactggattcacctcaaatcggtggcggtgcctctcttccaagtagtctgcgtctccatagagtttcctcatgactgagttcttggtctggaacagggttctcctcttgcccagcctcatggttccgcccatctgccctgggttgtgttctggcatgtctacgaccacgggatgactggtcgtagggtcaaactctgtagaattggcatcttgccatcccagcacgtttcttgagaattcaaccactgccaactgcatccctaagcacacgcccaaaaaaggctttttctgattccgagcccaggcaattgcttggatttttccttctgttcctcgaacaccaaatcctcctggaaccagcactccatgagcactacagagcttctgccaagcttcgtggtagcgcacgggctcttcttgcgaggtgatgggctccaagtccgcagaatctatgtacttgatttccaatttgtggttgatggccagtgcagaatgctccagagccttaatgacagaggcataggagtctgagaacttcgtgtatttgcccacaagggcaatagagcaggtctccagcaagcgatcatatctgtcagccatctctttccatttcatcagcatttttcttggctgcctctcaataggaaggtcaagtcttcgaagaaaataatctacaaccccttgctcctctaacaacaaggggactcggtagatggatgagacatcgtggacacagatcacttgttcaggctcaacatggcagaacattgatattttctccttcactgatgtgtcaagtggatttgagcacctgcatacaaccagatctggggaaagcccaagtcctctaagttcccgaacactattctgggtaggtttagtcttctgttcccctgttgaacttggctggggaactagactgacgtggatgttacaaaagttctctcttttgaccttgaattggaactgacggaaggcctcaataaagggcatgctttctatgtcccccacggttccaccaagctcaataacacacacttgaggttccaggccatcttcatctacaggtattaacgcctgtctcatcacccactcctggattgcatctgtgatatgagggacaacttggacagttttccccaagtaatctcctttccgttccttgttaatgacatactggtatatctttccagtggtcagattattgtccttggtgaggcggatgtcaaggaaccgctcatagttacccaggtcaaggtctacttccccaccatcatccagcacaaaaacctcaccatgctcataaggagagaatgttcctgcatcaatgttaatgtaggggtcaattttgattgaagttacatgtaaaccacatgacttgagtattgtgcccacactgctggcaatgattccttttccaattcctgatataacaccaccagtaaccagaatgtacttcattttactctttgacctaggggaatgggggtgagaatctctgcgccgcccgcgtcacagggccgctgaggattcgaaactgtaacgagcgtggacggaagggcgccacgcaaacgtggtgagctctatacaccgccagcgccccgacccccggccgccgggaagggaggaagccgtgaggcccaaaggccagccgcggggcccagggccggcgagttcgcaggccccctcgtcctacggcgcggagctgccgcgcccagccccgggcggctgagcccgcgccgaggccggaggcccgaggcccgcactgcttgaatggatgggcgactgccgggcttcctcgcagacgaagagcaagggcggagggtgtgggggggggcgccgctccactcccctacggccttctccgtccgacgagcccggccgagctgattcggcgcggcccagcgcggcagcgcaggccccgcagcctctgaagccgccccgcgccccgcttggcccctctccccagcgccgcccggccacgaggcccgcgcgcggg

SEQ ID NO: 8851 - RNA, 1850 nt, Homo sapiens
  source 1..1850: mol_type = other RNA
aatcctttgtccctgggtgagagcctgcagcctttctggaggtaatgtgagagccgccccacagaggccaggaggaggccaaagtatggtggggagggcttgataggcctggacaggaactcagggtggtactgaaccccaacaaaaaagggatgatcttctaactccacaatttccattctctctccttcaacatcttggccaacaaacttcaagccttgttcttccaaacactttttccagactggattcacctcaaatcggtggcggtgcctctcttccaagtagtctgcgtctccatagagtttcctcatgactgagttcttggtctggaacagggttctcctcttgcccagcctcatggttccgcccatctgccctgggttgtgttctggcatgtctacgaccacgggatgactggtcgtagggtcaaactctgtagaattggcatcttgccatcccagcacgtttcttgagaattcaaccactgccaactgcatccctaagcacacgcccaaaaaaggctttttctgattccgagcccaggcaattgcttggatttttccttctgttcctcgaacaccaaatcctcctggaaccagcactccatgagcactacagagcttctgccaagcttcgtggtagcgcacgggctcttcttgcgaggtgatgggctccaagtccgcagaatctatgtacttgatttccaatttgtggttgatggccagtgcagaatgctccagagccttaatgacagaggcataggagtctgagaacttcgtgtatttgcccacaagggcaatagagcaggtctccagcaagcgatcatatctgtcagccatctctttccatttcatcagcatttttcttggctgcctctcaataggaaggtcaagtcttcgaagaaaataatctacaaccccttgctcctctaacaacaaggggactcggtagatggatgagacatcgtggacacagatcacttgttcaggctcaacatggcagaacattgatattttctccttcactgatgtgtcaagtggatttgagcacctgcatacaaccagatctggggaaagcccaagtcctctaagttcccgaacactattctgggtaggtttagtcttctgttcccctgttgaacttggctggggaactagactgacgtggatgttacaaaagttctctcttttgaccttgaattggaactgacggaaggcctcaataaagggcatgctttctatgtcccccacggttccaccaagctcaataacacacacttgaggttccaggccatcttcatctacaggtattaacgcctgtctcatcacccactcctggattgcatctgtgatatgagggacaacttggacagttttccccaagtaatctcctttccgttccttgttaatgacatactggtatatctttccagtggtcagattattgtccttggtgaggcggatgtcaaggaaccgctcatagttacccaggtcaaggtctacttccccaccatcatccagcacaaaaacctcaccatgctcataaggagagaatgttcctgcatcaatgttaatgtaggggtcaattttgattgaagttacatgtaaaccacatgacttgagtattgtgcccacactgctggcaatgattccttttccaattcctgatataacaccaccagtaaccagaatgtacttcattttactctttgacctgcggccggcttcagatcctcccgtcagcgacagagctgggccggcgacgcgcgcggagccccggacagccagtgaacaaccccgaccgcatgcgcccggcagtctttcacggaggcgggctctaggctgtgc

SEQ ID NO: 8852 - RNA, 1848 nt, Homo sapiens
  source 1..1848: mol_type = other RNA
aatcctttgtccctgggtgagagcctgcagcctttctggaggtaatgtgagagccgccccacagaggccaggaggaggccaaagtatggtggggagggcttgataggcctggacaggaactcagggtggtactgaaccccaacaaaaaagggatgatcttctaactccacaatttccattctctctccttcaacatcttggccaacaaacttcaagccttgttcttccaaacactttttccagactggattcacctcaaatcggtggcggtgcctctcttccaagtagtctgcgtctccatagagtttcctcatgactgagttcttggtctggaacagggttctcctcttgcccagcctcatggttccgcccatctgccctgggttgtgttctggcatgtctacgaccacgggatgactggtcgtagggtcaaactctgtagaattggcatcttgccatcccagcacgtttcttgagaattcaaccactgccaactgcatccctaagcacacgcccaaaaaaggctttttctgattccgagcccaggcaattgcttggatttttccttctgttcctcgaacaccaaatcctcctggaaccagcactccatgagcactacagagcttctgccaagcttcgtggtagcgcacgggctcttcttgcgaggtgatgggctccaagtccgcagaatctatgtacttgatttccaatttgtggttgatggccagtgcagaatgctccagagccttaatgacagaggcataggagtctgagaacttcgtgtatttgcccacaagggcaatagagcaggtctccagcaagcgatcatatctgtcagccatctctttccatttcatcagcatttttcttggctgcctctcaataggaaggtcaagtcttcgaagaaaataatctacaaccccttgctcctctaacaacaaggggactcggtagatggatgagacatcgtggacacagatcacttgttcaggctcaacatggcagaacattgatattttctccttcactgatgtgtcaagtggatttgagcacctgcatacaaccagatctggggaaagcccaagtcctctaagttcccgaacactattctgggtaggtttagtcttctgttcccctgttgaacttggctggggaactagactgacgtggatgttacaaaagttctctcttttgaccttgaattggaactgacggaaggcctcaataaagggcatgctttctatgtcccccacggttccaccaagctcaataacacacacttgaggttccaggccatcttcatctacaggtattaacgcctgtctcatcacccactcctggattgcatctgtgatatgagggacaacttggacagttttccccaagtaatctcctttccgttccttgttaatgacatactggtatatctttccagtggtcagattattgtccttggtgaggcggatgtcaaggaaccgctcatagttacccaggtcaaggtctacttccccaccatcatccagcacaaaaacctcaccatgctcataaggagagaatgttcctgcatcaatgttaatgtaggggtcaattttgattgaagttacatgtaaaccacatgacttgagtattgtgcccacactgctggcaatgattccttttccaattcctgatataacaccaccagtaaccagaatgtacttcattttactctttgactttggcatggtcaggacattttcctcctcaggaacgttccatgtgaagccaaattatgataaaaataaactaaggaacaagaaaactaaggagttgtgctcgaagcattcccccgccccaccccctccccag

SEQ ID NO: 8853 - RNA, 1929 nt, Homo sapiens
  source 1..1929: mol_type = other RNA
aatcctttgtccctgggtgagagcctgcagcctttctggaggtaatgtgagagccgccccacagaggccaggaggaggccaaagtatggtggggagggcttgataggcctggacaggaactcagggtggtactgaaccccaacaaaaaagggatgatcttctaactccacaatttccattctctctccttcaacatcttggccaacaaacttcaagccttgttcttccaaacactttttccagactggattcacctgttgaggcatgaaaaataattctgctggtctctcagctcactatctttccagagtaccagcaagctggaatcctcacctcaaatcggtggcggtgcctctcttccaagtagtctgcgtctccatagagtttcctcatgactgagttcttggtctggaacagggttctcctcttgcccagcctcatggttccgcccatctgccctgggttgtgttctggcatgtctacgaccacgggatgactggtcgtagggtcaaactctgtagaattggcatcttgccatcccagcacgtttcttgagaattcaaccactgccaactgcatccctaagcacacgcccaaaaaaggctttttctgattccgagcccaggcaattgcttggatttttccttctgttcctcgaacaccaaatcctcctggaaccagcactccatgagcactacagagcttctgccaagcttcgtggtagcgcacgggctcttcttgcgaggtgatgggctccaagtccgcagaatctatgtacttgatttccaatttgtggttgatggccagtgcagaatgctccagagccttaatgacagaggcataggagtctgagaacttcgtgtatttgcccacaagggcaatagagcaggtctccagcaagcgatcatatctgtcagccatctctttccatttcatcagcatttttcttggctgcctctcaataggaaggtcaagtcttcgaagaaaataatctacaaccccttgctcctctaacaacaaggggactcggtagatggatgagacatcgtggacacagatcacttgttcaggctcaacatggcagaacattgatattttctccttcactgatgtgtcaagtggatttgagcacctgcatacaaccagatctggggaaagcccaagtcctctaagttcccgaacactattctgggtaggtttagtcttctgttcccctgttgaacttggctggggaactagactgacgtggatgttacaaaagttctctcttttgaccttgaattggaactgacggaaggcctcaataaagggcatgctttctatgtcccccacggttccaccaagctcaataacacacacttgaggttccaggccatcttcatctacaggtattaacgcctgtctcatcacccactcctggattgcatctgtgatatgagggacaacttggacagttttccccaagtaatctcctttccgttccttgttaatgacatactggtatatctttccagtggtcagattattgtccttggtgaggcggatgtcaaggaaccgctcatagttacccaggtcaaggtctacttccccaccatcatccagcacaaaaacctcaccatgctcataaggagagaatgttcctgcatcaatgttaatgtaggggtcaattttgattgaagttacatgtaaaccacatgacttgagtattgtgcccacactgctggcaatgattccttttccaattcctgatataacaccaccagtaaccagaatgtacttcattttactctttgacctgcggccggcttcagatcctcccgtcagcgacagagctgggccggcgacgcgcgcggagccccggacagccagtgaacaaccccgaccgcatgcgcccggcagtctttcacggaggcgggctctaggctgtgc

SEQ ID NO: 8854 - RNA, 1365 nt, Homo sapiens
  source 1..1365: mol_type = other RNA
aatgcacctgggcaaggattcactttctggcaaggcatgccaagtagctgtatcctcctcttcactgctggactcctcatccaatcgggtccacaaaagaggggatgagcaggagtctagaggactctggggaggactctgcggaggaccctggggagagatcttgggaggaccctggggaggaatctcaggaggactctggggaagaggtggcatcccagcagcaggcatatcctcatcttctcctcccttcttctgttgtggggacgcctcggtcagccctcggcggccatcttcctgtctgtggcctgcaagtccttgaggattggccaggtctaagacgcttccctctgctgacctgagtccagactcctcgcaaaatgcttcaggtccttcagactcccacagtgcaagtcgggaaagcacatccgcgaaccctgccaaggctgaccagggccctattgcattcagcacttcccagatgacctcctcagatgcacagttgccctttatgaagatcacactcagaataagaatcaggaggcggttctggggcatgccctgctcatcactcagactcccctcacaggtgaggtctaatgtgtttacaaagacatagaaatggtcggggtccacttctgtcagggaaatgccaaaaagaatctctatgaactcacgggctttcctgaagatcataggaaagtagcccgtgtatgtgttgatgacattcatctgcatctctgctcttgtgagaggctcttttgcttgatatttgaggagaagaaactgcaccaacttgtccaccttttcatccagtgtataagtgaacaagggctcgctctctggcaagctccccgctttctccccccacaacctttttccagggctgacggcaggaagggaaagggtgtagcctgtgcctctcctccatgttggaaggtcactgtccttccacagagttctcttctcgttgagtggccagtcctggggttcctccctctgcttaactgaaactgccctcctcagagaaaacttcccctccggctgactcccaaaatgcaagtcagaaagttgtaaacctggggaccctgatagggtcctccagagcttgaagtatgtggggcagaggacaagactatccattcgctgatctgaagttccacccctcagaaaaagcctcacctccctcagatgcccaagatgaaaggcagaatagtccttatctgtggcctttttccggggctggggctgaggtgggagcaccactggggataaggcatatgtggcacatgtgtttttcacccactggcctagactgccatcactgaaggtggcatccaacacccagtggcagggcagcagcat

SEQ ID NO: 8855 - RNA, 998 nt, Homo sapiens
  source 1..998: mol_type = other RNA
aatgcacctgggcaaggattcactttctggcaaggcatgccaagtagctgtatcctcctcttcactgctggactcctcatccaatcgggtccacaaaagaggggatgagcaggagtctagaggactctggggaggactctgcggaggaccctggggagagatcttgggaggaccctggggaggaatctcaggaggactctggggaagaggtggcatcccagcagcaggcatatcctcatcttctggaacacccagaatgagagtagagggtaagggtgaggacaagggtgaggatgaggacaaggaagaggaggaggggaataaaaagtggaaagaggaagaggaagtggaggaggcatcctcctcctcctcatctatggaatcctgtgcatctaccaagtcctctgtcacactcgggttctggaagtcttcctcaaagctgaggcgtggaaggtttggaaagagaggcatgaggcctgttgttcaggagcagcaggtaaacgtgtgagcagggatggggatgatgggatcccacaggcagctcttcttctcttaaggtggtgctctagggcctcacaggtcgcctgtcttcctaagaggtttgctccctcagaaccttgactcctgatattgcctgggcctcctctgctgtgctgactttaggaagtgtgcctcagacccaggtcttcaactcctggttcctggagcaccttgaggattggccaggtctaagacgcttccctctgctgacctgagtccagactcctcgcaaaatgcttcaggtccttcagactcccacagtgcaagtcgggaaagcacatccgcgaaccctgccaaggctgaccagggctctccgttttcacctctccatctgttttgtccaggggtgacagcaaggagtggctgggcgacgcctgggccttccctccgtgttgggagatagctatccttccacagagttcccttcttgcttgttggccagccccggggctcctttc

SEQ ID NO: 8856 - RNA, 1892 nt, Homo sapiens
  source 1..1892: mol_type = other RNA
aatgcacctgggcaaggattcactttctggcaaggcatgccaagtagctgtatcctcctcttcactgctggactcctcatccaatcgggtccacaaaagaggggatgagcaggagtctagaggactctggggaggactctgcggaggaccctggggagagatcttgggaggaccctggggaggaatctcaggaggactctggggaagaggtggcatcccagcagcaggcatatcctcatcttctggaacacccagaatgagagtagagggtaagggtgaggacaagggtgaggatgaggacaaggaagaggaggaggggaataaaaagtggaaagaggaagaggaagtggaggaggcatcctcctcctcctcatctatggaatcctgtgcatctaccaagtcctctgtcacactcgggttctggaagtcttcctcaaagctgaggcgtggaaggtttggaaagagaggcatgaggcctgttgttcaggagcagcaggtaaacgtgtgagcagggatggggatgatgggatcccacaggcagctcttcttctcttaaggtggtgctctagggcctcacaggtcgcctgtcttcctaagaggtttgctccctcagaaccttgactcctgatattgcctgggcctcctctgctgtgctgactttaggaagtgtgcctcagacccaggtcttcaactcctggttcctggagcaccttgaggattggccaggtctaagacgcttccctctgctgacctgagtccagactcctcgcaaaatgcttcaggtccttcagactcccacagtgcaagtcgggaaagcacatccgcgaaccctgccaaggctgaccagggctctccgttttcacctctccatctgttttgtccaggggtgacagcaaggagtggctgggcgacgcctgggccttccctccgtgttgggagatagctatccttccacagagttcccttcttgcttgttggccagccccggggctcctttctctgcttaactgaagctgccccgtgtccatggtggttctgacaaaggccggcttacagctcttcttctcttaaggtggtgctctagggcctcacgggtcacctgccatcctagggggtttgtcccctgggaaccttgactcctgatattgcctgggcctcctctgctgtgctgactttaggaagtgtgcctcagacccaggtcttcaactcctggttcctggagcacctgcaagaggaagtgagggagcccctcaggctaaagactgcaagcagagtcttgggcctcccaaggctgacagctggggctgaccagactcccagagccccacagttctggactgcatggtcccatcagaatttaattagcatcctcaccttttctcagacagggccatgtccctaccactcttctagccaaaactcagggcaaactccacatccctgagagcagtgggaggtagtgaggtggcagccacctcccagcactctaccacgggggcagttgggctggcctcacatctgttctgatgcacatgtgactcctcagtcctcactcttatccccagcagggcctgggaatcttccctctgccaactggaggcagctccctgtgctgatttgccacgggaccctcagaccaaggccttccctttccctgcacctctcacccagcaatgagagggctgccgctcagcctgagctgactggggagctctacgagggctgatatggaggagcatgctgggaatctctgggagtctgtcctctgaggtggcgtttccccttgtccttctcaaagtcttcctatttattccctagagagctggcacctcctcccttcttctgtcatgaagacgtgtccctcagccctcggttaccctcttcctgtctgc

SEQ ID NO: 8857 - RNA, 834 nt, Homo sapiens
  source 1..834: mol_type = other RNA
aatgcacctgggcaaggattcactttctggcaaggcatgccaagtagctgtatcctcctcttcactgctggactcctcatccaatcgggtccacaaaagaggggatgagcaggagtctagaggactctggggaggactctgcggaggaccctggggagagatcttgggaggaccctggggaggaatctcaggaggactctggggaagaggtggcatcccagcagcaggcatatcctcatcttctggaacacccagaatgagagtagagggtaagggtgaggacaagggtgaggatgaggacaaggaagaggaggaggggaataaaaagtggaaagaggaagaggaagtggaggaggcatcctcctcctcctcatctatggaatcctgtgcatctaccaagtcctctgtcacactcgggttctggaagtcttcctcaaagctgaggcgtggaaggtttggaaagagaggcatgaggcctgttgttcaggagcagcaggtaaacgtgtgagcagggatggggatgatgggatcccacaggccttgactcctgatattgcctgggcctcctctgctgtgctgactttaggaagtgtgcctcagacccaggtcttcaactcctggttcctggagcaccttgaggattggccaggtctaagacgcttccctctgctgacctgagtccagactcctcgcaaaatgcttcaggtccttcagactcccacagtgcaagtcgggaaagcacatccgcgaaccctgccaaggctgaccagggctgacagcagaggcagcgtggggtggggcctcctctccatggaaaaaccaccccccacctct

SEQ ID NO: 8858 - RNA, 25 nt, Homo sapiens
  source 1..25: mol_type = other RNA
aatgtggactggtgtgaccaaatgt

SEQ ID NO: 8859 - RNA, 2821 nt, Homo sapiens
  source 1..2821: mol_type = other RNA
aatgttttttcctgtttccatttgttgccggcgttggtaaggcctggactctcgccacaggaattctcattttctgctgggctcctgtccttgatgcatctgtttcgacagcagctgcactggaacctgtgtcctgagcaggtgcatcagatgaactcagcttccgagtaactttcccagccactttatctgacatgggtcttacttgccgacgaagagccgtaacatctcttttacgttgatcctttttcaactgagcaatctctctgtttcttctagactcagtcagtctggctttctcttgttcttctttcatttgtttcattaggcgaacctttgtttttttcatttccatcacatcctgctgcaatttcttcaattgcttttcatactgagactgatttttaagcaaccttgcatgttctttttgagctgcttgaagtctctgcagttctttgttcatggcttggagtttcttttcatattcagacctaactttttttgctttttcttctgagtaagattctaccgagcctaagttttgaagcacctggtctctttcaagctgagtatcccgaattttatgttgcagcatcattagcttctcttcatactgctttttcagagtctgcagtcttttctggctgttttctagttcatcaatcagcttttgcttaattgcaatttcacaagtaatgtttgccaagtctgcttgataattggctttttcatctgattcagaatctgattcatcagaactttcacccccatcaatgtcatcttcctcctcctcctcctcctcttcttcatcctcatgatcactcacttcttgactttcttccacttctaattcattgttttctctttccgaaacacccttttcttctttcttctcttggtcagtgtctgtattatcctctttaccagccacacttctttcttctcgattgctttcctcaagtttctgtagcctttttttcttcctcttttcttttcttttcaacttctctaaatctttttttgctaggtctataatttcaatggtttctttgtctgaggatagtatggtaggagaaaaagttgatgatccgctgaaatatggcgctcttgctgtggctcttgtcaagttttttcgaaggttctcattcactgcttcactttctaataattttgccctgagatcttcgatttcttttatataactatgaatcatattactaatctcctcatttccttcacctgctctggcaagaacatggttggcctgatcactaacaagctgtgtaattctggacctcaatgcatcaaccgtctcttgcatggctttaattcttacacgcaggttattattttcagtctgtagcatagcattctcatgaaacatgtcattgatgctttccacaccctcttcgtcaattattcttttacctgttttgtactccatgagctccatctgaagtcgtgtgatttcactacgaagtgcattgatttgctgactagctctgtcctgattgaccatcaccttattcttgatatttctagctcgattggcgtatttcagggtgtttaacgtttccataaagtctctgtctgaagggctgacacatgctatcatgattgtttggctattacccccgagggaatcctgtagtagtcttgttagcttggaatctctataggggacatgtgtggccctcttgctcttgtctcccaaggcacttattacattgccaagtgccaaaagtccacagttgatagaaatgccttcttttgccctctcgcctgtagctccagtacgcttcagtctttcagatcctgcgagatcaacaaaatggaactttgcagtcagggtttcaaattcattcatctgtgctgattcagaaataattttattatcagttgcattgtcagcatctatttggggacacactctggtttgacacacatgaatggtaaaaatggcatgtgaacgagagctctgaacattcatctgggtactggcagttgtccgggataaagcacccaacttcaaacactgcatcatctctgattctgtattcacagtacgtgttgtaacgcccacagtataaattcctccagttgaatcttcatgaattcttatatttgattttttactttttgcatcaatatcacgagtggtatcaaataagtcaaggacctcttcattatagagctctaagaattgggcattcactttaaaatctggagcaggaagcccatttttaattgctatgtgttttttttcttcaatactcttaaaaaggtgtttaacagctcgagaaataatacccagttcttcctcaacaatgttaacatcaaatcctgttcccattgtgtatgttttaccagctccagtttgtccataagcaaaaactgtagcattgtatccttcaaagcaaccttcaattagtttttctatacattgaatgtagatctgctcttgctgggagtcaatgtcaaatacatagtcaaaagtaaaagccttatctttccctaggaagacctgaggctctcctggtgtgacagatgtacaaatatggcatccttcaatcttctctttggcaagctgtggtcttattctgacagccacccgcacggagctctcgtccggggcgcccaacatgctggcggcgggcagcgatcgagccgttgggcctcggcaccgcagagctgaggcgccactggggccgcgggactcgggcgcagtaggctggggcgtctgcgggcgggcggccggctcacctccgccgcgctccagccatgttgggcgactgaatggaaaggtggcggcggcgctgag

SEQ ID NO: 8860 - RNA, 2755 nt, Homo sapiens
  source 1..2755: mol_type = other RNA
aatgttttttcctgtttccatttgttgccggcgttggtaaggcctggactctcgccacaggaattctcattttctgctgggctcctgtccttgatgcatctgtttcgacagcagctgcactggaacctgtgtcctgagcaggtgcatcagatgaactcagcttccgagtaactttcccagccactttatctgacatgggtcttacttgccgacgaagagccgtaacatctcttttacgttgatcctttttcaactgagcaatctctctgtttcttctagactcagtcagtctggctttctcttgttcttctttcatttgtttcattaggcgaacctttgtttttttcatttccatcacatcctgctgcaatttcttcaattgcttttcatactgagactgatttttaagcaaccttgcatgttctttttgagctgcttgaagtctctgcagttctttgttcatggcttggagtttcttttcatattcagacctaactttttttgctttttcttctgagtaagattctaccgagcctaagttttgaagcacctggtctctttcaagctgagtatcccgaattttatgttgcagcatcattagcttctcttcatactgctttttcagagtctgcagtcttttctggctgttttctagttcatcaatcagcttttgcttaattgcaatttcacaagtaatgtttgccaagtctgcttgataattggctttttcatctgattcagaatctgattcatcagaactttcacccccatcaatgtcatcttcctcctcctcctcctcctcttcttcatcctcatgatcactcacttcttgactttcttccacttctaattcattgttttctctttccgaaacacccttttcttctttcttctcttggtcagtgtctgtattatcctctttaccagccacactttttttcttcctcttttcttttcttttcaacttctctaaatctttttttgctaggtctataatttcaatggtttctttgtctgaggatagtatggtaggagaaaaagttgatgatccgctgaaatatggcgctcttgctgtggctcttgtcaagttttttcgaaggttctcattcactgcttcactttctaataattttgccctgagatcttcgatttcttttatataactatgaatcatattactaatctcctcatttccttcacctgctctggcaagaacatggttggcctgatcactaacaagctgtgtaattctggacctcaatgcatcaaccgtctcttgcatggctttaattcttacacgcaggttattattttcagtctgtagcatagcattctcatgaaacatgtcattgatgctttccacaccctcttcgtcaattattcttttacctgttttgtactccatgagctccatctgaagtcgtgtgatttcactacgaagtgcattgatttgctgactagctctgtcctgattgaccatcaccttattcttgatatttctagctcgattggcgtatttcagggtgtttaacgtttccataaagtctctgtctgaagggctgacacatgctatcatgattgtttggctattacccccgagggaatcctgtagtagtcttgttagcttggaatctctataggggacatgtgtggccctcttgctcttgtctcccaaggcacttattacattgccaagtgccaaaagtccacagttgatagaaatgccttcttttgccctctcgcctgtagctccagtacgcttcagtctttcagatcctgcgagatcaacaaaatggaactttgcagtcagggtttcaaattcattcatctgtgctgattcagaaataattttattatcagttgcattgtcagcatctatttggggacacactctggtttgacacacatgaatggtaaaaatggcatgtgaacgagagctctgaacattcatctgggtactggcagttgtccgggataaagcacccaacttcaaacactgcatcatctctgattctgtattcacagtacgtgttgtaacgcccacagtataaattcctccagttgaatcttcatgaattcttatatttgattttttactttttgcatcaatatcacgagtggtatcaaataagtcaaggacctcttcattatagagctctaagaattgggcattcactttaaaatctggagcaggaagcccatttttaattgctatgtgttttttttcttcaatactcttaaaaaggtgtttaacagctcgagaaataatacccagttcttcctcaacaatgttaacatcaaatcctgttcccattgtgtatgttttaccagctccagtttgtccataagcaaaaactgtagcattgtatccttcaaagcaaccttcaattagtttttctatacattgaatgtagatctgctcttgctgggagtcaatgtcaaatacatagtcaaaagtaaaagccttatctttccctaggaagacctgaggctctcctggtgtgacagatgtacaaatatggcatccttcaatcttctctttggcaagctgtggtcttattctgacagccacccgcacggagctctcgtccggggcgcccaacatgctggcggcgggcagcgatcgagccgttgggcctcggcaccgcagagctgaggcgccactggggccgcgggactcgggcgcagtaggctggggcgtctgcgggcgggcggccggctcacctccgccgcgctccagccatgttgggcgact

SEQ ID NO: 8861 - RNA, 2863 nt, Homo sapiens
  source 1..2863: mol_type = other RNA
aatgttttttcctgtttccatttgttgccggcgttggtaaggcctggactctcgccacaggaattctcattttctgctgggctcctgtccttgatgcatctgtttcgacagcagctgcactggaacctgtgtcctgagcaggtgcatcagatgaactcagcttccgagtaactttcccagccactttatctgacatgggtcttacttgccgacgaagagccgtaacctcttcagttttgcgacgtagaaccacttcttggtttcttttttgggcttccagaagtctaagttgatgatctcttttacgttgatcctttttcaactgagcaatctctctgtttcttctagactcagtcagtctggctttctcttgttcttctttcatttgtttcattaggcgaacctttgtttttttcatttccatcacatcctgctgcaatttcttcaattgcttttcatactgagactgatttttaagcaaccttgcatgttctttttgagctgcttgaagtctctgcagttctttgttcatggcttggagtttcttttcatattcagacctaactttttttgctttttcttctgagtaagattctaccgagcctaagttttgaagcacctggtctctttcaagctgagtatcccgaattttatgttgcagcatcattagcttctcttcatactgctttttcagagtctgcagtcttttctggctgttttctagttcatcaatcagcttttgcttaattgcaatttcacaagtaatgtttgccaagtctgcttgataattggctttttcatctgattcagaatctgattcatcagaactttcacccccatcaatgtcatcttcctcctcctcctcctcctcttcttcatcctcatgatcactcacttcttgactttcttccacttctaattcattgttttctctttccgaaacacccttttcttctttcttctcttggtcagtgtctgtattatcctctttaccagccacacttctttcttctcgattgctttcctcaagtttctgtagcctttttttcttcctcttttcttttcttttcaacttctctaaatctttttttgctaggtctataatttcaatggtttctttgtctgaggatagtatggtaggagaaaaagttgatgatccgctgaaatatggcgctcttgctgtggctcttgtcaagttttttcgaaggttctcattcactgcttcactttctaataattttgccctgagatcttcgatttcttttatataactatgaatcatattactaatctcctcatttccttcacctgctctggcaagaacatggttggcctgatcactaacaagctgtgtaattctggacctcaatgcatcaaccgtctcttgcatggctttaattcttacacgcaggttattattttcagtctgtagcatagcattctcatgaaacatgtcattgatgctttccacaccctcttcgtcaattattcttttacctgttttgtactccatgagctccatctgaagtcgtgtgatttcactacgaagtgcattgatttgctgactagctctgtcctgattgaccatcaccttattcttgatatttctagctcgattggcgtatttcagggtgtttaacgtttccataaagtctctgtctgaagggctgacacatgctatcatgattgtttggctattacccccgagggaatcctgtagtagtcttgttagcttggaatctctataggggacatgtgtggccctcttgctcttgtctcccaaggcacttattacattgccaagtgccaaaagtccacagttgatagaaatgccttcttttgccctctcgcctgtagctccagtacgcttcagtctttcagatcctgcgagatcaacaaaatggaactttgcagtcagggtttcaaattcattcatctgtgctgattcagaaataattttattatcagttgcattgtcagcatctatttggggacacactctggtttgacacacatgaatggtaaaaatggcatgtgaacgagagctctgaacattcatctgggtactggcagttgtccgggataaagcacccaacttcaaacactgcatcatctctgattctgtattcacagtacgtgttgtaacgcccacagtataaattcctccagttgaatcttcatgaattcttatatttgattttttactttttgcatcaatatcacgagtggtatcaaataagtcaaggacctcttcattatagagctctaagaattgggcattcactttaaaatctggagcaggaagcccatttttaattgctatgtgttttttttcttcaatactcttaaaaaggtgtttaacagctcgagaaataatacccagttcttcctcaacaatgttaacatcaaatcctgttcccattgtgtatgttttaccagctccagtttgtccataagcaaaaactgtagcattgtatccttcaaagcaaccttcaattagtttttctatacattgaatgtagatctgctcttgctgggagtcaatgtcaaatacatagtcaaaagtaaaagccttatctttccctaggaagacctgaggctctcctggtgtgacagatgtacaaatatggcatccttcaatcttctctttggcaagctgtggtcttattctgacagccacccgcacggagctctcgtccggggcgcccaacatgctggcggcgggcagcgatcgagccgttgggcctcggcaccgcagagctgaggcgccactggggccgcgggactcgggcgcagtaggctggggcgtctgcgggcgggcggccggctcacctccgccgcgctccagccatgttgggcgact

SEQ ID NO: 8862 - RNA, 2890 nt, Homo sapiens
  source 1..2890: mol_type = other RNA
aatgttttttcctgtttccatttgttgccggcgttggtaaggcctggactctcgccacaggaattctcattttctgctgggctcctgtccttgatgcatctgtttcgacagcagctgcactggaacctgtgtcctgagcaggtgcatcagatgaactcagcttccgagtaactttcccagccactttatctgacatgggtcttacttgccgacgaagagccgtaacctcttcagttttgcgacgtagaaccacttcttggtttcttttttgggcttccagaagtctaagttgatgatctcttttacgttgatcctttttcaactgagcaatctctctgtttcttctagactcagtcagtctggctttctcttgttcttctttcatttgtttcattaggcgaacctttgtttttttcatttccatcacatcctgctgcaatttcttcaattgcttttcatactgagactgatttttaagcaaccttgcatgttctttttgagctgcttgaagtctctgcagttctttgttcatggcttggagtttcttttcatattcagacctaactttttttgctttttcttctgagtaagattctaccgagcctaagttttgaagcacctggtctctttcaagctgagtatcccgaattttatgttgcagcatcattagcttctcttcatactgctttttcagagtctgcagtcttttctggctgttttctagttcatcaatcagcttttgcttaattgcaatttcacaagtaatgtttgccaagtctgcttgataattggctttttcatctgattcagaatctgattcatcagaactttcacccccatcaatgtcatcttcctcctcctcctcctcctcttcttcatcctcatgatcactcacttcttgactttcttccacttctaattcattgttttctctttccgaaacacccttttcttctttcttctcttggtcagtgtctgtattatcctctttaccagccacacttctttcttctcgattgctttcctcaagtttctgtagcctttttttcttcctcttttcttttcttttcaacttctctaaatctttttttgctaggtctataatttcaatggtttctttgtctgaggatagtatggtaggagaaaaagttgatgatccgctgaaatatggcgctcttgctgtggctcttgtcaagttttttcgaaggttctcattcactgcttcactttctaataattttgccctgagatcttcgatttcttttatataactatgaatcatattactaatctcctcatttccttcacctgctctggcaagaacatggttggcctgatcactaacaagctgtgtaattctggacctcaatgcatcaaccgtctcttgcatggctttaattcttacacgcaggttattattttcagtctgtagcatagcattctcatgaaacatgtcattgatgctttccacaccctcttcgtcaattattcttttacctgttttgtactccatgagctccatctgaagtcgtgtgatttcactacgaagtgcattgatttgctgactagctctgtcctgattgaccatcaccttattcttgatatttctagctcgattggcgtatttcagggtgtttaacgtttccataaagtctctgtctgaagggctgacacatgctatcatgattgtttggctattacccccgagggaatcctgtagtagtcttgttagcttggaatctctataggggacatgtgtggccctcttgctcttgtctcccaaggcacttattacattgccaagtgccaaaagtccacagttgatagaaatgccttcttttgccctctcgcctgtagctccagtacgcttcagtctttcagatcctgcgagatcaacaaaatggaactttgcagtcagggtttcaaattcattcatctgtgctgattcagaaataattttattatcagttgcattgtcagcatctatttggggacacactctggtttgacacacatgaatggtaaaaatggcatgtgaacgagagctctgaacattcatctgggtactggcagttgtccgggataaagcacccaacttcaaacactgcatcatctctgattctgtattcacagtacgtgttgtaacgcccacagtataaattcctccagttgaatcttcatgaattcttatatttgattttttactttttgcatcaatatcacgagtggtatcaaataagtcaaggacctcttcattatagagctctaagaattgggcattcactttaaaatctggagcaggaagcccatttttaattgctatgtgttttttttcttcaatactcttaaaaaggtgtttaacagctcgagaaataatacccagttcttcctcaacaatgttaacatcaaatcctgttcccattgtgtatgttttaccagctccagtttgtccataagcaaaaactgtagcattgtatccttcaaagcaaccttcaattagtttttctatacattgaatgtagatctgctcttgctgggagtcaatgtcaaatacatagtcaaaagtaaaagccttatctttccctaggaagacctgaggctctcctggtgtgacagatgtacaaatatggcatccttcaatcttctctttggcaagctgtggtcttattctgacagccacccgcacggagctctcgtccggggcgcccaacatgctggcggcgggcagcgatcgagccgttgggcctcggcaccgcagagctgaggcgccactggggccgcgggactcgggcgcagtaggctggggcgtctgcgggcgggcggccggctcacctccgccgcgctccagccatgttgggcgactgaatggaaaggtggcggcggcgctgag

SEQ ID NO: 8863 - RNA, 2824 nt, Homo sapiens
  source 1..2824: mol_type = other RNA
aatgttttttcctgtttccatttgttgccggcgttggtaaggcctggactctcgccacaggaattctcattttctgctgggctcctgtccttgatgcatctgtttcgacagcagctgcactggaacctgtgtcctgagcaggtgcatcagatgaactcagcttccgagtaactttcccagccactttatctgacatgggtcttacttgccgacgaagagccgtaacctcttcagttttgcgacgtagaaccacttcttggtttcttttttgggcttccagaagtctaagttgatgatctcttttacgttgatcctttttcaactgagcaatctctctgtttcttctagactcagtcagtctggctttctcttgttcttctttcatttgtttcattaggcgaacctttgtttttttcatttccatcacatcctgctgcaatttcttcaattgcttttcatactgagactgatttttaagcaaccttgcatgttctttttgagctgcttgaagtctctgcagttctttgttcatggcttggagtttcttttcatattcagacctaactttttttgctttttcttctgagtaagattctaccgagcctaagttttgaagcacctggtctctttcaagctgagtatcccgaattttatgttgcagcatcattagcttctcttcatactgctttttcagagtctgcagtcttttctggctgttttctagttcatcaatcagcttttgcttaattgcaatttcacaagtaatgtttgccaagtctgcttgataattggctttttcatctgattcagaatctgattcatcagaactttcacccccatcaatgtcatcttcctcctcctcctcctcctcttcttcatcctcatgatcactcacttcttgactttcttccacttctaattcattgttttctctttccgaaacacccttttcttctttcttctcttggtcagtgtctgtattatcctctttaccagccacactttttttcttcctcttttcttttcttttcaacttctctaaatctttttttgctaggtctataatttcaatggtttctttgtctgaggatagtatggtaggagaaaaagttgatgatccgctgaaatatggcgctcttgctgtggctcttgtcaagttttttcgaaggttctcattcactgcttcactttctaataattttgccctgagatcttcgatttcttttatataactatgaatcatattactaatctcctcatttccttcacctgctctggcaagaacatggttggcctgatcactaacaagctgtgtaattctggacctcaatgcatcaaccgtctcttgcatggctttaattcttacacgcaggttattattttcagtctgtagcatagcattctcatgaaacatgtcattgatgctttccacaccctcttcgtcaattattcttttacctgttttgtactccatgagctccatctgaagtcgtgtgatttcactacgaagtgcattgatttgctgactagctctgtcctgattgaccatcaccttattcttgatatttctagctcgattggcgtatttcagggtgtttaacgtttccataaagtctctgtctgaagggctgacacatgctatcatgattgtttggctattacccccgagggaatcctgtagtagtcttgttagcttggaatctctataggggacatgtgtggccctcttgctcttgtctcccaaggcacttattacattgccaagtgccaaaagtccacagttgatagaaatgccttcttttgccctctcgcctgtagctccagtacgcttcagtctttcagatcctgcgagatcaacaaaatggaactttgcagtcagggtttcaaattcattcatctgtgctgattcagaaataattttattatcagttgcattgtcagcatctatttggggacacactctggtttgacacacatgaatggtaaaaatggcatgtgaacgagagctctgaacattcatctgggtactggcagttgtccgggataaagcacccaacttcaaacactgcatcatctctgattctgtattcacagtacgtgttgtaacgcccacagtataaattcctccagttgaatcttcatgaattcttatatttgattttttactttttgcatcaatatcacgagtggtatcaaataagtcaaggacctcttcattatagagctctaagaattgggcattcactttaaaatctggagcaggaagcccatttttaattgctatgtgttttttttcttcaatactcttaaaaaggtgtttaacagctcgagaaataatacccagttcttcctcaacaatgttaacatcaaatcctgttcccattgtgtatgttttaccagctccagtttgtccataagcaaaaactgtagcattgtatccttcaaagcaaccttcaattagtttttctatacattgaatgtagatctgctcttgctgggagtcaatgtcaaatacatagtcaaaagtaaaagccttatctttccctaggaagacctgaggctctcctggtgtgacagatgtacaaatatggcatccttcaatcttctctttggcaagctgtggtcttattctgacagccacccgcacggagctctcgtccggggcgcccaacatgctggcggcgggcagcgatcgagccgttgggcctcggcaccgcagagctgaggcgccactggggccgcgggactcgggcgcagtaggctggggcgtctgcgggcgggcggccggctcacctccgccgcgctccagccatgttgggcgact

SEQ ID NO: 8864 - RNA, 2851 nt, Homo sapiens
  source 1..2851: mol_type = other RNA
aatgttttttcctgtttccatttgttgccggcgttggtaaggcctggactctcgccacaggaattctcattttctgctgggctcctgtccttgatgcatctgtttcgacagcagctgcactggaacctgtgtcctgagcaggtgcatcagatgaactcagcttccgagtaactttcccagccactttatctgacatgggtcttacttgccgacgaagagccgtaacctcttcagttttgcgacgtagaaccacttcttggtttcttttttgggcttccagaagtctaagttgatgatctcttttacgttgatcctttttcaactgagcaatctctctgtttcttctagactcagtcagtctggctttctcttgttcttctttcatttgtttcattaggcgaacctttgtttttttcatttccatcacatcctgctgcaatttcttcaattgcttttcatactgagactgatttttaagcaaccttgcatgttctttttgagctgcttgaagtctctgcagttctttgttcatggcttggagtttcttttcatattcagacctaactttttttgctttttcttctgagtaagattctaccgagcctaagttttgaagcacctggtctctttcaagctgagtatcccgaattttatgttgcagcatcattagcttctcttcatactgctttttcagagtctgcagtcttttctggctgttttctagttcatcaatcagcttttgcttaattgcaatttcacaagtaatgtttgccaagtctgcttgataattggctttttcatctgattcagaatctgattcatcagaactttcacccccatcaatgtcatcttcctcctcctcctcctcctcttcttcatcctcatgatcactcacttcttgactttcttccacttctaattcattgttttctctttccgaaacacccttttcttctttcttctcttggtcagtgtctgtattatcctctttaccagccacactttttttcttcctcttttcttttcttttcaacttctctaaatctttttttgctaggtctataatttcaatggtttctttgtctgaggatagtatggtaggagaaaaagttgatgatccgctgaaatatggcgctcttgctgtggctcttgtcaagttttttcgaaggttctcattcactgcttcactttctaataattttgccctgagatcttcgatttcttttatataactatgaatcatattactaatctcctcatttccttcacctgctctggcaagaacatggttggcctgatcactaacaagctgtgtaattctggacctcaatgcatcaaccgtctcttgcatggctttaattcttacacgcaggttattattttcagtctgtagcatagcattctcatgaaacatgtcattgatgctttccacaccctcttcgtcaattattcttttacctgttttgtactccatgagctccatctgaagtcgtgtgatttcactacgaagtgcattgatttgctgactagctctgtcctgattgaccatcaccttattcttgatatttctagctcgattggcgtatttcagggtgtttaacgtttccataaagtctctgtctgaagggctgacacatgctatcatgattgtttggctattacccccgagggaatcctgtagtagtcttgttagcttggaatctctataggggacatgtgtggccctcttgctcttgtctcccaaggcacttattacattgccaagtgccaaaagtccacagttgatagaaatgccttcttttgccctctcgcctgtagctccagtacgcttcagtctttcagatcctgcgagatcaacaaaatggaactttgcagtcagggtttcaaattcattcatctgtgctgattcagaaataattttattatcagttgcattgtcagcatctatttggggacacactctggtttgacacacatgaatggtaaaaatggcatgtgaacgagagctctgaacattcatctgggtactggcagttgtccgggataaagcacccaacttcaaacactgcatcatctctgattctgtattcacagtacgtgttgtaacgcccacagtataaattcctccagttgaatcttcatgaattcttatatttgattttttactttttgcatcaatatcacgagtggtatcaaataagtcaaggacctcttcattatagagctctaagaattgggcattcactttaaaatctggagcaggaagcccatttttaattgctatgtgttttttttcttcaatactcttaaaaaggtgtttaacagctcgagaaataatacccagttcttcctcaacaatgttaacatcaaatcctgttcccattgtgtatgttttaccagctccagtttgtccataagcaaaaactgtagcattgtatccttcaaagcaaccttcaattagtttttctatacattgaatgtagatctgctcttgctgggagtcaatgtcaaatacatagtcaaaagtaaaagccttatctttccctaggaagacctgaggctctcctggtgtgacagatgtacaaatatggcatccttcaatcttctctttggcaagctgtggtcttattctgacagccacccgcacggagctctcgtccggggcgcccaacatgctggcggcgggcagcgatcgagccgttgggcctcggcaccgcagagctgaggcgccactggggccgcgggactcgggcgcagtaggctggggcgtctgcgggcgggcggccggctcacctccgccgcgctccagccatgttgggcgactgaatggaaaggtggcggcggcgctgag

SEQ ID NO: 8865 - RNA, 254 nt, Homo sapiens
  source 1..254: mol_type = other RNA
aatgttttttcctgtttcccaagactttcaaaatgaggtaacacctccacggcctggcccgcgggacccgccagctcgaccaacaacggcctgcagccgcacctccgcaagctcctcttttccttctcagctctcggagaggggcagtgtcgcgtcaggagggccggaaaacggccccgcagcgctgccctcggggggtccgcctcctgaactggccacttcccgcagcagccgcggctccttccggtgtctcc

SEQ ID NO: 8866 - RNA, 108 nt, Homo sapiens
  source 1..108: mol_type = other RNA
aatgttttttcctgtttcccaagactttcaaaatgaggtaacacctttaaggttaatatcgttatgtgtgaatttgatcctgtcattacgatgttagctggttatttt

SEQ ID NO: 8867 - RNA, 433 nt, Homo sapiens
  source 1..433: mol_type = other RNA
aatgttttttcctgtttcccaagactttcaaaatgaggtaacacctttaaggttaatatcgttatgtgtgaatttgatcctgtcattacgatgttagctggttattttgctcattagttgaggcagtttcttcctaacatcgatggtctttacaatttggcatgtttttgcagtggctggtaccggttgttcctttccatgtttagtgcttccttcaggagctctccacggcctggcccgcgggacccgccagctcgaccaacaacggcctgcagccgcacctccgcaagctcctcttttccttctcagctctcggagaggggcagtgtcgcgtcaggagggccggaaaacggccccgcagcgctgccctcggggggtccgcctcctgaactggccacttcccgcagcagccgcggctccttccggtgtctcc

SEQ ID NO: 8868 - RNA, 2119 nt, Homo sapiens
  source 1..2119: mol_type = other RNA
aattctgtaaaggaagaagaggcaggtgagaaaggtgggaacttatggaagaaagggaagaacaaatgctaatatcaataaagcccctcctgggaaccaagccctgcaataggcccctttcccaacatgctctttgaggtctcttgaccgcattcatggatgatatggcagagcccagaactgagcaaagtcactctaccttcacaccgaggaagagctggagagatgctgggggcaatctctgcatgatgactgcatgctggttatatccaacaaggctgcattgcaagggaggagtgattcaaaaggacccagcaccagctaatgactgttaccgaaatgagttcctgaaaccatggggaaatgaaatcaacagtccaccaagtccagaaacccggcccaaagggctagatctgttccttacttgctccgaagccatagcagctgccttttctgtaaaatggggacaatttctcagggttgttccatggattatataggacagcatttatgaaagaaagacatcgtaaattatataataatactcaactgcaataactaatggttctgcctccatatttgggtcttggattaatgtcttcctctgccggtgacaaaccgagaagcaggaaaagaagattctctgagttgatcaggcaatggcaggttttccagtgattgaacacccacccacttccacctccccacctcacccgctacctgggccctgggggcctgggcattcttgcccttccactgtactgcacacagcaggagcttcattcccggatgagccccaggtcagacactggctgggctggacccatgagtcagggctctgcggcagactgaatcaacagagaagacaggcctggcccagccagtggcccaaacagaaagggaaaggccaatgcctttgcttggtctgggctgggccggggctgtaacagttgtaggcagaagctgagttcaagctgggggtaaataaatacatctccagcaaagcagaaggaagcacatgtgttgtttggtgacctctcaacttcctccttccctctattaactccaggttaagacaattctatccgacctctgttttctcatctgaaaataaggaagttgccttgtttcagctttgcatcttctgatcatggcggggacccaccatggtgatggggtctggctggatctctgaattttacctggtacccacatctctcagacccattctctcctttccttagctcaggattgttgcttctgggctcagaggagatgcagctggccataagtccctatttctatcctgctcagggatgtcatcgacattgatggcccccagttgacactcacaggcctaaaatgcacctacctccctgcccatgagccccagtactcgtgaccttctgcagctcctcttccaaaggtgtatctgtccatcagctctgacctgtctgtgtcacagatatttgccaaagagcttcaagaaaagccaaagaatgagctactcatggggaaactcaggcagcacaacagtaagggcagagcatggtgaggacatgagtttgacctcctcaagccactcagcatagccaggtgatggcttttttatgttttccttgagccttgggtgcatagcattgggggaactagaatccttgcttcatgacttttttcactattggtccatgcagggcccatttgtaacttgctagttagttggatttaacaatgtaataagcctccataaacccatcatccccaacaaaagctggacttaatagtaacctacatctaaccatgaggttcccactcctgcacacacatatccatccctctcctgaggtgggtagagcaagtgtctttcgtttattaattcgacaaatattggctatacatatttgataggcagggactgtactacaagctccctgcccaagtaagttcttcccaaaccccatattcatcattcccttgcttctctatagaaaagattctgtgctatatgtaatcttttgggactaagtttttcccttaatattacattctaatatcatccttattattattttgagatggagtgttgctctgtcccccaggctggagtgctgtggcacca

SEQ ID NO: 8869 - RNA, 29 nt, Homo sapiens
  source 1..29: mol_type = other RNA
aatttactctgcaatcttctccaattgct

SEQ ID NO: 8870 - RNA, 2504 nt, Homo sapiens
  source 1..2504: mol_type = other RNA
acaaggtgtgcatgcctgacccatccatagctaatacatttcttgtgtgtggatgcctggcgaaagtccccaggggctcttcgggcaggcatttgctctttgggcagagaaggaagttgggctttgagagactacgcagtattttagggactagctaaagtgcagttccaggtcctatgagggaggtgacaccataatcccattttacagaaggggatgctgaggcccttgggtatcagtggcttactccaggtcacatggctaggaaggggtgagggccgattcctgagcctgctcttccatgctccactgccgtacctcacccaggtacccaagcatgcctgcgatgcttcaagaacacagctggcggcatgcgtatcttcactgctagatagcgaagccgcacactaggccggctccaggatctagcccagggcagttcacacgcataaatctgctcaggaggaaccagtgcctcccaagacatgatgccaagggccttagtgatccacaagtggcaggtgaatgacaaccaaagggagagggaaggctgtgtaaggcaggtggccatggagacagggggcatagcactgatggaggagggcagagggggagggtaaaccaggcctgtgcccaaaaaagcacatggtggtgatgatggagacgctggtatgttacagaaaacagggcgcccttcagaggggctgctgtgggtggagctggatcgtggaagtcctgaggaacgtggacttggggactgaaggcaaaggggagcccggctggcttgtgagcagcagacagtagtgattgcaactggcacatcgtggctggactggagaggggtgcacaggacaccctgtgggagtctagagagtggcccggtctccatgagcatgacttgggaagtccgtttcctttggagcctgtttccctgctcctttctgcatcggcgcctgcccatttgccccacagcccagcagtgccagcaggttgggagaacccttcgatgtgcttgcaaatcttcctctttgcaccttagtgcctcctgcttgttcctttgctggggaagtcggggaaaaaaaagattctgctgaagcacaaatagtggctcagagtaggcagtgtggagaagtgccccagagaaacacgattaaccaggattagggtcacatgagaaggaggcgaatatgttttcatattcatagcctcacaaaaagaatttaaatccacaaatcttcttatgtgtgtggatcgaggagtgctacatttggagtcctaggatagccaaatgacattagaagcgtgtaacgtggctgggaattccaggggttgcactatgcgcgcacccaggctcacacctgtcccagaagaaaggatttccccccatttgggtggtgctggaggctgataaagaagagacaattcagagctcctaatgccccttacacctgccctcaggcatctgtcgctggttctaaaaccctcagcataaaggaagggctggaggtgtggccgctctggagccgagattcacagtctgacacgtggcttaaagaggcccctttctccctagtccgtgacttcacggaaatattttaatgctactgattttcaggggcatccaggaggtgcctgaaggagctgaggggcagcctctagcagtgtccctaatggggattaagatcacgttataaacccagctactacaatggcgaggcatgcagcaccctccagggttccgggatgggtgggagcgtcaggcgacagcaggcatttcgcatgaaccatcccatccctacacactgaaggttggaggggtgtcacggtgtccagttggatcacaggattaaactgccctggcccaggctcagccccacccccatacctgggccccagaggagaggaagagtagctctcatcagaaagggcccagcagtcaggaaaggagggagaccttgccctcttgaccaggggctgccaagctgtccagtgggaggagcgaaaacatgggtggccggagcatatgggcaaggatcggcaccacggggtcagggcatgctcagagcagctgaggcctggcagccctggtgaggctcgggatggacgatacgaggggacactgggcagcttggaccagcagaggcccagcaagcaggtgggagaacagaggccagttctgaccaggaggcattcccagagcctgtccctgggggtcaggaggcgtggaccatggagagactgagatactagtattgatgtctccccaagtgcacccccagctcatgagtcctggagatggctggggaagaaagcactgggtcctgtccctaaagtgcaccaactctgtgccaggctccaagtcagcacttctcttaggttgcttgtttgacctcaacagctttaccaaggggtggtatgttctctttcaaagtgaagaaatggggccaggcgtggtggctcaagcctgtaatcctagcactttgggaggctgcagcaggtggatc

SEQ ID NO: 8871 - RNA, 2086 nt, Homo sapiens
  source 1..2086: mol_type = other RNA
acaaggtgtgcatgcctgaccctaggcacttttcacctatatcctgtcgctttttccccaggcttctagtcttttaggcacccattcacagatctcaaagatgtattggggaaagcaatttgattaaactagtttacgttaaaatatgaatgacaacacagagcttcattttttaaaaagcccttataaatacaacataaactgaaattggtggacttataagcagtattaatagaaaatatttcagatagttaaagtatgtttggtcaattaaaatgccactgttatctaaactgtttgtttcatttgattagcacttatgcgcttctcaacactgagaagacatattcagtgctaaccttaagtattttacattgactttcaaggcacaggcaatgaggggagaaaagttgaggcttgttacaagtggtcatatatgagctcttcaaaaatttaatgtaagtcaggaatactttaagtctcaaatatcatcagaatgtggcagcagtgggtgagtagtgtattagaaagggcacagcctggggtcaagtggactctgcctgggtggcttggggtaggtttaacctcacagcttttttaatctattaaacaaggttttggtatctattttatagggtagtgatgaggattaaacgagatgatgtatataaattgtttagcacctagtaaatgctcaataaataatgcagctaatattagttattattttatagtaacaacagcaaatataataatagacaccagatatgaatctgacaagaccaaaaagaaatgataaagaaatgactaagataaggaaaatgattttattgattttagtgtggctcagatatctttgaatgttccctttactctcaaataaggagattcaagtagcacaaatctaaaaggaaaaatgaaatttagaggaaaaaaatttatgaatcttaaggggatatgaagattttttttaattaaaggagactggaacataatatgtgatgaaaaatcacaaaccaaattactgaaattaagaaattatgctatcatggttgacattaaaggtgactggtccttgatgaagtgattaatagacatgcatatgggtgtgggtgttttcaaagaaatactcattaatagtgatgacataaatggacctgacaactaagaccacgtttataaaaggcaagttttaaaatgtagattagatagccttatatatattatcaagaagaaacatgacaatacatgaatttagatataatgtagacatgaagaaataagagttatgttttaattttacagcagtgatagaaacaaaatacttggggaaaagtatttttcttagggagaaaaattgagctgctgttagtatgtaactcagcccagtaacatgatgaggtggatagagccaggctttgtgcctgctacaggaagagctgctgcagcgtcagttctcaagctaccaagaaaacctagtattcatgtaaaacagacgtcattatgcatgtgtaagatggaatcctctgataaatagaacaagaggattctaataggcatgatcttgtgaacgcagtctcagggagtacaataagatgttttaaatagaaagtaatgaatgaagcattcttctttggaataagcaatctactgtttcatgaacagaagttgggttcagattttcaaaaaaatgcctgctaggcatagtctaacagatatccagcagaatggttttctatttttgaattagaattaagatcacttactcatgattttcaactcgagccaagtcaagtaatcttatcttgtactgatgaagatgtcagagactatgccagtggctgtacctggatttcttcaatgaaacacatcacttctataaacgcttattttactttttcatattttcctattattttatttatttcttcatgcctcagcaagcagataacttcaggtcctatagcagaatcccaagagaaatatctggaaatcagtgaacctgcaaagcccttgggggttccagtgtatatttgttgtcatcaggaatctgggtgtggtggctggtgcctgtaatcccagctag

SEQ ID NO: 8872 - RNA, 31 nt, Homo sapiens
  source 1..31: mol_type = other RNA
acacatgggtggctgtggcctaaacactgcc

SEQ ID NO: 8873 - RNA, 559 nt, Homo sapiens
  source 1..559: mol_type = other RNA
acacatgggtggctgtggcctgcgccaccagctgcatatgcacgtacttgatggttccatctgcgttgcgctcctgcagcaggaagtagtagccatcctcctgagggtgctcgtcctgtgcccgccggggccatagcagcacccggtgcacaggcgagtcgttggcgtccagcacccattcctcgcctcccgactctttgacctccaccagcacataacatttggtgccgtccagccgcaggctggcaatggcgtccttgatgacgtccgaggtggtgctgtccttggtggcagtcacgcggcacgaggcctggctctcggtggtggacagctgggggtagatgtgcaggtggtaggccgcctgctcccggcggcccgagctgcctgcctctttcacactcatcctgccggccgcctggcttcagcatgcctcccaggctcggggcgcgcgtgtcctggagctggcctcggccgccgcgcgccgccggtcccgggccgggtccccggccggacgaccgcctgccagcccgccgctgctcgagccgctccgccccgccgc

SEQ ID NO: 8874 - RNA, 152 nt, Homo sapiens
  source 1..152: mol_type = other RNA
acactgtccccttctccccagcacgttctcttctctccctggtttatttttctccacagcacttatcatcatcagatcacataaatttcactgtcttctcatcccacttgaacctgaagcaccagctatactcaggaggctgaggtgggagg

SEQ ID NO: 8875 - RNA, 52 nt, Homo sapiens
  source 1..52: mol_type = other RNA
acactgtccccttctccccagctgtcctcgcagagcctccagccaagcggcc

SEQ ID NO: 8876 - RNA, 2895 nt, Homo sapiens
  source 1..2895: mol_type = other RNA
acactgtccccttctccccagggctgtatgggagcacaggcacaggggtaggtagagcttctggtcagcgaggggtagagcccacagagagaccagagagtggaccgcagtttcatgaaagcagagttatagctgccacttgtgcctgtgggcagagcaggtggtagaggggcctccaggaaagggccggggacacgggtgtccagcactaagcacagcgcactcagccgcagcctctgtctgtctccccacccgcccacctctggcacacagcacctggggacccagatttgtgcttgatcagagcttcgaaggaaggcagtggcagaggcgctgggaggctgtcctggaagtggccaattctggtgtcctctgcaaagtacccctcgtccctggacaaccagaacgtgccctgacctcttccctggcccgtccccacccgcggtgtgtgatccttagacgtgagtctgcatccgccgctgcaggggtcgactggggtcagagttctgggacgaggactgggagtggtgggaggaggaagcagaagccttgctggccttgtcgaactgcacatagccatcctgcttgccgctgctgctgacgctgctgtcacactgcgtgtccaggaaggagctgctgtcgctgagggagcctctctggaactcccgctcacaaagctcgatggacgagctgcccatgcccagcacaaaccgctgcccgtagtcgtagaggcggccctggccgctcagggtgctgtagatgttggtgaaggacatgcctgtgggcacacgctgcttgcccgcaggacgcaggtcgggctggcagctggagagggagatggtcggggttgagtggtgctctttgaaggtgttgacgctgtagtagccattggtggggtccttcaggttctgaaactctttctcctcttctttgaggacctccagctgtttcaggactgagtcttgctggaattcaccccggtccatcatcagctgcttgatggtggagtgctcctcaccctcccgaccagaggctggttccttgtggacaatttccactcggatatcatttttggctgacacaacacctttgagatttctctgggaacgggcacagcagaacgccacgatggttgccataaggacgaggaaggccacaccagctcctacggccaccccaatgatgacggccatcggcacagactctgcttccagcccggctcccgacttcatttccgaaccttgctccttgagccggatgatctcagtgtcggagccgaagctgttccaggccgtgcagttgtagatggtctggaagtcggcccgcacgatgttgctgatggtcagggtggagatgacgccctcctcggtgctgatggtctccaccgtatagcgccccgatgtgcccgactccagaacgttctccttccaggaccaggcgatgcggtccggcggcggcgtgctccggatgaagcacttgatctggcccttctcgccgtggagggcgtgctgggtctgggtgctggagatgatggggggtccattgacggtcagggtcacctctctctccccggctcccacacggggcaccacagcccggcacacgtacttgcccgcgtcctcctggcgcacggatttgagggtcagggtcttctcattgctcaggaccactccggagccccgcttcatccagacgatggtcagggatgggttgccggtccaggcgcagctgaagatggcatcagagcccagatccacgagcaaggattggggttctgtggtcatccggggcccaaagtagacgtcaaccgtgcggctgaggttggtgctgcccagggcgttggtcacctcacaggagacgggctctgagaagtacgtgtagtccactgtggtcctgtacacctctccagatgcctccttgatgatctggccccgcttggcccacctgtactgggtgacagctgggttggcctttgcagagcagtggaaagtgacgacgttgtcctccagcactggctgtggctccaccgagaggttgaccagtggagggtgctggatgtcaatggtgaccgacgtctcctttcctccggggatggctttgttggtggcacgacacacgatgctctggccattctccacgtcaccaggggagatgaagagggtgctgacgatgctctcccgcttgccgtcccgaagcagggtcttggagtaggtggccccattgatgacctctccctttcgcaaccagatgatggaggctgcaggcttggcattgtctgcgtggcaggtgaggttgagagggtcccccgcacgcaggctgatcacagggccccccaggatgacggggtcatcaggcggcaccaggactgtgaggcgtgcggggcgggagcggatggcggcctggatggcctggcactcgtacaccgcatcgtcttgcagctctgccctcaggatcttcaggtggtgctcccctgacaggtggttccctaccaccaggtactgtgggtaacttgagaggtccctgcccacacccagagccaagccgtccttgatccacagaacgaagccatcgtattcggggatggcgcaaagtagcgtcactggctgtcccgacaccaccacctggtcctggggctgctggctgaaggaatagacttggccttcattcattctccgaaacttgtccttggccatgtagcccagcaccagacagcatcctctcttctggaggcccagctcattttgttgcattcgcaaaggcgaagaggcaatgccagagcatctcagcccggcaccgagagacgcatccatcagtccgagttcccgaagcctgcccacgttcctgcccacagcctcccgcgccctgacaacccagccgactttcttccaactccag

SEQ ID NO: 8877 - RNA, 3053 nt, Homo sapiens
  source 1..3053: mol_type = other RNA
acactgtccccttctccccagggctgtatgggagcacaggcacaggggtaggtagagcttctggtcagcgaggggtagagcccacagagagaccagagagtggaccgcagtttcatgaaagcagagttatagctgccacttgtgcctgtgggcagagcaggtggtagaggggcctccaggaaagggccggggacacgggtgtccagcactaagcacagcgcactcagccgcagcctctgtctgtctccccacccgcccacctctggcacacagcacctggggacccagatttgtgcttgatcagagcttcgaaggaaggcagtggcagaggcgctgggaggctgtcctggaagtggccaattctggtgtcctctgcaaagtacccctcgtccctggacaaccagaacgtgccctgacctcttccctggcccgtccccacccgcggtgtgtgatccttagacgtgagtctgcatccgccgctgcaggggtcgactggggtcagagttctgggacgaggactgggagtggtgggaggaggaagcagaagccttgctggccttgtcgaactgcacatagccatcctgcttgccgctgctgctgacgctgctgtcacactgcgtgtccaggaaggagctgctgtcgctgagggagcctctctggaactcccgctcacaaagctcgatggacgagctgcccatgcccagcacaaaccgctgcccgtagtcgtagaggcggccctggccgctcagggtgctgtagatgttggtgaaggacatgcctgtgggcacacgctgcttgcccgcaggacgcaggtcgggctggcagctggagagggagatggtcggggttgagtggtgctctttgaaggtgttgacgctgtagtagccattggtggggtccttcaggttctgaaactctttctcctcttctttgaggacctccagctgtttcaggactgagtcttgctggaattcaccccggtccatcatcagctgcttgatggtggagtgctcctcaccctcccgaccagaggctggttccttgtggacaatttccactcggatatcatttttggctgacacaacacctttgagatttctctgggaacgggcacagcagaacgccacgatggttgccataaggacgaggaaggccacaccagctcctacggccaccccaatgatgacggccatcggcacagactctgcttccagcccggctcccgacttcatttccgaaccttgctccttgagccggatgatctcagtgtcggagccgaagctgttccaggccgtgcagttgtagatggtctggaagtcggcccgcacgatgttgctgatggtcagggtggagatgacgccctcctcggtgctgatggtctccaccgtatagcgccccgatgtgcccgactccagaacgttctccttccaggaccaggcgatgcggtccggcggcggcgtgctccggatgaagcacttgatctggcccttctcgccgtggagggcgtgctgggtctgggtgctggagatgatggggggtccattgacggtcagggtcacctctctctccccggctcccacacggggcaccacagcccggcacacgtacttgcccgcgtcctcctggcgcacggatttgagggtcagggtcttctcattgctcaggaccactccggagccccgcttcatccagacgatggtcagggatgggttgccggtccaggcgcagctgaagatggcatcagagcccagatccacgagcaaggattggggttctgtggtcatccggggcccaaagtagacgtcaaccgtgcggctgaggttggtgctgcccagggcgttggtcacctcacaggagacgggctctgagaagtacgtgtagtccactgtggtcctgtacacctctccagatgcctccttgatgatctggccccgcttggcccacctgtactgggtgacagctgggttggcctttgcagagcagtggaaagtgacgacgttgtcctccagcactggctgtggctccaccgagaggttgaccagtggagggtgctggatgtcaatggtgaccgacgtctcctttcctccggggatggctttgttggtggcacgacacacgatgctctggccattctccacgtcaccaggggagatgaagagggtgctgacgatgctctcccgcttgccgtcccgaagcagggtcttggagtaggtggccccattgatgacctctccctttcgcaaccagatgatggaggctgcaggcttggcattgtctgcgtggcaggtgaggttgagagggtcccccgcacgcaggctgatcacagggccccccaggatgacggggtcatcaggcggcaccaggactgtgaggcgtgcggggcgggagcggatggcggcctggatggcctggcactcgtacaccgcatcgtcttgcagctctgccctcaggatcttcaggtggtgctcccctgacaggtggttccctaccaccaggtactgtgggtaacttgagaggtccctgcccacacccagagccaagccgtccttgatccacagaacgaagccatcgtattcggggatggcgcaaagtagcgtcactggctgtcccgacaccaccacctggtcctggggctgctggctgaaggaatagacttggccttcattcattctccgaaacttgtccttggccatgtagcccagcaccagacagcatcctctcttctggaggcccagctcttgactgaagaggaagaagcagacgaagagcagatcgagctggaagggtttcattccttagcgcagcgaaggaaagccggcggggtaacttggctgtggttagtttctcttccttggcggctctcggtgctcagcctccgccggtcctctcgggttcgcgcctaccatctgtccgtccgtgggtccctccgggtggcttcggtctctttgtgcctctgggtatctgcagccagccgacacaaactgcctgttcttagccgcctcgggaagccgggattgtcagcaatgtccccactcggagaagatccattctct

SEQ ID NO: 8878 - RNA, 3217 nt, Homo sapiens
  source 1..3217: mol_type = other RNA
acactgtccccttctccccagggctgtatgggagcacaggcacaggggtaggtagagcttctggtcagcgaggggtagagcccacagagagaccagagagtggaccgcagtttcatgaaagcagagttatagctgccacttgtgcctgtgggcagagcaggtggtagaggggcctccaggaaagggccggggacacgggtgtccagcactaagcacagcgcactcagccgcagcctctgtctgtctccccacccgcccacctctggcacacagcacctggggacccagatttgtgcttgatcagagcttcgaaggaaggcagtggcagaggcgctgggaggctgtcctggaagtggccaattctggtgtcctctgcaaagtacccctcgtccctggacaaccagaacgtgccctgacctcttccctggcccgtccccacccgcggtgtgtgatccttagacgtgagtctgcatccgccgctgcaggggtcgactggggtcagagttctgggacgaggactgggagtggtgggaggaggaagcagaagccttgctggccttgtcgaactgcacatagccatcctgcttgccgctgctgctgacgctgctgtcacactgcgtgtccaggaaggagctgctgtcgctgagggagcctctctggaactcccgctcacaaagctcgatggacgagctgcccatgcccagcacaaaccgctgcccgtagtcgtagaggcggccctggccgctcagggtgctgtagatgttggtgaaggacatgcctgtgggcacacgctgcttgcccgcaggacgcaggtcgggctggcagctggagagggagatggtcggggttgagtggtgctctttgaaggtgttgacgctgtagtagccattggtggggtccttcaggttctgaaactctttctcctcttctttgaggacctccagctgtttcaggactgagtcttgctggaattcaccccggtccatcatcagctgcttgatggtggagtgctcctcaccctcccgaccagaggctggttccttgtggacaatttccactcggatatcatttttggctgacacaacacctttgagatttctctgggaacgggcacagcagaacgccacgatggttgccataaggacgaggaaggccacaccagctcctacggccaccccaatgatgacggccatcggcacagactctgcttccagcccggctcccgacttcatttccgaaccttgctccttgagccggatgatctcagtgtcggagccgaagctgttccaggccgtgcagttgtagatggtctggaagtcggcccgcacgatgttgctgatggtcagggtggagatgacgccctcctcggtgctgatggtctccaccgtatagcgccccgatgtgcccgactccagaacgttctccttccaggaccaggcgatgcggtccggcggcggcgtgctccggatgaagcacttgatctggcccttctcgccgtggagggcgtgctgggtctgggtgctggagatgatggggggtccattgacggtcagggtcacctctctctccccggctcccacacggggcaccacagcccggcacacgtacttgcccgcgtcctcctggcgcacggatttgagggtcagggtcttctcattgctcaggaccactccggagccccgcttcatccagacgatggtcagggatgggttgccggtccaggcgcagctgaagatggcatcagagcccagatccacgagcaaggattggggttctgtggtcatccggggcccaaagtagacgtcaaccgtgcggctgaggttggtgctgcccagggcgttggtcacctcacaggagacgggctctgagaagtacgtgtagtccactgtggtcctgtacacctctccagatgcctccttgatgatctggccccgcttggcccacctgtactgggtgacagctgggttggcctttgcagagcagtggaaagtgacgacgttgtcctccagcactggctgtggctccaccgagaggttgaccagtggagggtgctggatgtcaatggtgaccgacgtctcctttcctccggggatggctttgttggtggcacgacacacgatgctctggccattctccacgtcaccaggggagatgaagagggtgctgacgatgctctcccgcttgccgtcccgaagcagggtcttggagtaggtggccccattgatgacctctccctttcgcaaccagatgatggaggctgcaggcttggcattgtctgcgtggcaggtgaggttgagagggtcccccgcacgcaggctgatcacagggccccccaggatgacggggtcatcaggcggcaccaggactgtgaggcgtgcggggcgggagcggatggcggcctggatggcctggcactcgtacaccgcatcgtcttgcagctctgccctcaggatcttcaggtggtgctcccctgacaggtggttccctaccaccaggtactgtgggtaacttgagaggtccctgcccacacccagagccaagccgtccttgatccacagaacgaagccatcgtattcggggatggcgcaaagtagcgtcactggctgtcccgacaccaccacctggtcctggggctgctggctgaaggaatagacttggccttcattcattctccgaaacttgtccttggccatgtagcccagcaccagacagcatcctctcttctggaggcccagctcttgactgaagaggaagaagcagacgaagagcagatcgagctggaagggtttcattccttagcgcagcgaaggaaagccggcggggtaacttggctgtggttagtttctcttccttggcggctctcggtgctcagcctccgccggtcctctcgggttcgcgcctaccatctgtccgtccgtgggtccctccgggtggcttcggtctctttgtgcctctgggtatctgcagccagccgacacaaactgcctgttcttagccgcctcgggaagccgggattgtcagcaatgtccccactcggagaagatccattctctggctcttggcatcccaggcacacggcttcctcaggcgggctcctcccacagtgagcgagcgagctagtgacgagtgacagaaggactcctttcactgaagctcctccgggggctcggttagcctcctggcgctgcaaggctgcctgcgcgcggttcgctccggg

SEQ ID NO: 8879 - RNA, 3352 nt, Homo sapiens
  source 1..3352: mol_type = other RNA
acactgtccccttctccccagggctgtatgggagcacaggcacaggggtaggtagagcttctggtcagcgaggggtagagcccacagagagaccagagagtggaccgcagtttcatgaaagcagagttatagctgccacttgtgcctgtgggcagagcaggtggtagaggggcctccaggaaagggccggggacacgggtgtccagcactaagcacagcgcactcagccgcagcctctgtctgtctccccacccgcccacctctggcacacagcacctggggacccagatttgtgcttgatcagagcttcgaaggaaggcagtggcagaggcgctgggaggctgtcctggaagtggccaattctggtgtcctctgcaaagtacccctcgtccctggacaaccagaacgtgccctgacctcttccctggcccgtccccacccgcggtgtgtgatccttagacgtgagtctgcatccgccgctgcaggggtcgactggggtcagagttctgggacgaggactgggagtggtgggaggaggaagcagaagccttgctggccttgtcgaactgcacatagccatcctgcttgccgctgctgctgacgctgctgtcacactgcgtgtccaggaaggagctgctgtcgctgagggagcctctctggaactcccgctcacaaagctcgatggacgagctgcccatgcccagcacaaaccgctgcccgtagtcgtagaggcggccctggccgctcagggtgctgtagatgttggtgaaggacatgcctgtgggcacacgctgcttgcccgcaggacgcaggtcgggctggcagctggagagggagatggtcggggttgagtggtgctctttgaaggtgttgacgctgtagtagccattggtggggtccttcaggttctgaaactctttctcctcttctttgaggacctccagctgtttcaggactgagtcttgctggaattcaccccggtccatcatcagctgcttgatggtggagtgctcctcaccctcccgaccagaggctggttccttgtggacaatttccactcggatatcatttttggctgacacaacacctttgagatttctctgggaacgggcacagcagaacgccacgatggttgccataaggacgaggaaggccacaccagctcctacggccaccccaatgatgacggccatcggcacagactctgcttccagcccggctcccgacttcatttccgaaccttgctccttgagccggatgatctcagtgtcggagccgaagctgttccaggccgtgcagttgtagatggtctggaagtcggcccgcacgatgttgctgatggtcagggtggagatgacgccctcctcggtgctgatggtctccaccgtatagcgccccgatgtgcccgactccagaacgttctccttccaggaccaggcgatgcggtccggcggcggcgtgctccggatgaagcacttgatctggcccttctcgccgtggagggcgtgctgggtctgggtgctggagatgatggggggtccattgacggtcagggtcacctctctctccccggctcccacacggggcaccacagcccggcacacgtacttgcccgcgtcctcctggcgcacggatttgagggtcagggtcttctcattgctcaggaccactccggagccccgcttcatccagacgatggtcagggatgggttgccggtccaggcgcagctgaagatggcatcagagcccagatccacgagcaaggattggggttctgtggtcatccggggcccaaagtagacgtcaaccgtgcggctgaggttggtgctgcccagggcgttggtcacctcacaggagacgggctctgagaagtacgtgtagtccactgtggtcctgtacacctctccagatgcctccttgatgatctggccccgcttggcccacctgtactgggtgacagctgggttggcctttgcagagcagtggaaagtgacgacgttgtcctccagcactggctgtggctccaccgagaggttgaccagtggagggtgctggatgtcaatggtgaccgacgtctcctttcctccggggatggctttgttggtggcacgacacacgatgctctggccattctccacgtcaccaggggagatgaagagggtgctgacgatgctctcccgcttgccgtcccgaagcagggtcttggagtaggtggccccattgatgacctctccctttcgcaaccagatgatggaggctgcaggcttggcattgtctgcgtggcaggtgaggttgagagggtcccccgcacgcaggctgatcacagggccccccaggatgacggggtcatcaggcggcaccaggactgtgaggcgtgcggggcgggagcggatggcggcctggatggcctggcactcgtacaccgcatcgtcttgcagctctgccctcaggatcttcaggtggtgctcccctgacaggtggttccctaccaccaggtactgtgggtaacttgagaggtccctgcccacacccagagccaagccgtccttgatccacagaacgaagccatcgtattcggggatggcgcaaagtagcgtcactggctgtcccgacaccaccacctggtcctggggctgctggctgaaggaatagacttggccttcattcattctccgaaacttgtccttggccatgtagcccagcaccagacagcatcctctcttctggaggcccagctcttgactgaagaggaagaagcagacgaagagcagatcgagctggaagggtttcattccttagcgcagcgaaggaaagccggcggggtaacttggctgtggttagtttctcttccttggcggctctcggtgctcagcctccgccggtcctctcgggttcgcgcctaccatctgtccgtccgtgggtccctccgggtggcttcggtctctttgtgcctctgggtatctgcagccagccgacacaaactgcctgttcttagccgcctcgggaagccgggattgtcagcaatgtccccactcggagaagatccattctctggctcttggcatcccaggcacacggcttcctcaggcgggctcctcccacagtgagcgagcgagctagtgacgagtgacagaaggactcctttcactgaagctgcaggacccacagccggtcgggctctggcgccagcctcgacggcggccccgccatctccgcccggctgcccgcggcctcacctcctccgggggctcggttagcctcctggcgctgcaaggctgcctgcgcgcggttcgctccgggggagggaggaggagggaggcggcgaggagccgacggctccacctgatggaga

SEQ ID NO: 8880 - RNA, 2859 nt, Homo sapiens
  source 1..2859: mol_type = other RNA
acactgtccccttctccccagggctgtatgggagcacaggcacaggggtaggtagagcttctggtcagcgaggggtagagcccacagagagaccagagagtggaccgcagtttcatgaaagcagagttatagctgccacttgtgcctgtgggcagagcaggtggtagaggggcctccaggaaagggccggggacacgggtgtccagcactaagcacagcgcactcagccgcagcctctgtctgtctccccacccgcccacctctggcacacagcacctggggacccagatttgtgcttgatcagagcttcgaaggaaggcagtggcagaggcgctgggaggctgtcctggaagtggccaattctggtgtcctctgcaaagtacccctcgtccctggacaaccagaacgtgccctgacctcttccctggcccgtccccacccgcggtgtgtgatccttagacgtgagtctgcatccgccgctgcaggggtcgactggggtcagagttctgggacgaggactgggagtggtgggaggaggaagcagaagccttgctggccttgtcgaactgcacatagccatcctgcttgccgctgctgctgacgctgctgtcacactgcgtgtccaggaaggagctgctgtcgctgagggagcctctctggaactcccgctcacaaagctcgatggacgagctgcccatgcccagcacaaaccgctgcccgtagtcgtagaggcggccctggccgctcagggtgctgtagatgttggtgaaggacatgcctgtgggcacacgctgcttgcccgcaggacgcaggtcgggctggcagctggagagggagatggtcggggttgagtggtgctctttgaaggtgttgacgctgtagtagccattggtggggtccttcaggttctgaaactctttctcctcttctttgaggacctccagctgtttcaggactgagtcttgctggaattcaccccggtccatcatcagctgcttgatggtggagtgctcctcaccctcccgaccagaggctggttccttgtggacaatttccactcggatatcatttttggctgacacaacacctttgagatttctctgggaacgggcacagcagaacgccacgatggttgccataaggacgaggaaggccacaccagctcctacggccaccccaatgatgacggccatcggcacagactcttgctccttgagccggatgatctcagtgtcggagccgaagctgttccaggccgtgcagttgtagatggtctggaagtcggcccgcacgatgttgctgatggtcagggtggagatgacgccctcctcggtgctgatggtctccaccgtatagcgccccgatgtgcccgactccagaacgttctccttccaggaccaggcgatgcggtccggcggcggcgtgctccggatgaagcacttgatctggcccttctcgccgtggagggcgtgctgggtctgggtgctggagatgatggggggtccattgacggtcagggtcacctctctctccccggctcccacacggggcaccacagcccggcacacgtacttgcccgcgtcctcctggcgcacggatttgagggtcagggtcttctcattgctcaggaccactccggagccccgcttcatccagacgatggtcagggatgggttgccggtccaggcgcagctgaagatggcatcagagcccagatccacgagcaaggattggggttctgtggtcatccggggcccaaagtagacgtcaaccgtgcggctgaggttggtgctgcccagggcgttggtcacctcacaggagacgggctctgagaagtacgtgtagtccactgtggtcctgtacacctctccagatgcctccttgatgatctggccccgcttggcccacctgtactgggtgacagctgggttggcctttgcagagcagtggaaagtgacgacgttgtcctccagcactggctgtggctccaccgagaggttgaccagtggagggtgctggatgtcaatggtgaccgacgtctcctttcctccggggatggctttgttggtggcacgacacacgatgctctggccattctccacgtcaccaggggagatgaagagggtgctgacgatgctctcccgcttgccgtcccgaagcagggtcttggagtaggtggccccattgatgacctctccctttcgcaaccagatgatggaggctgcaggcttggcattgtctgcgtggcaggtgaggttgagagggtcccccgcacgcaggctgatcacagggccccccaggatgacggggtcatcaggcggcaccaggactgtgaggcgtgcggggcgggagcggatggcggcctggatggcctggcactcgtacaccgcatcgtcttgcagctctgccctcaggatcttcaggtggtgctcccctgacaggtggttccctaccaccaggtactgtgggtaacttgagaggtccctgcccacacccagagccaagccgtccttgatccacagaacgaagccatcgtattcggggatggcgcaaagtagcgtcactggctgtcccgacaccaccacctggtcctggggctgctggctgaaggaatagacttggccttcattcattctccgaaacttgtccttggccatgtagcccagcaccagacagcatcctctcttctggaggcccagctcattttgttgcattcgcaaaggcgaagaggcaatgccagagcatctcagcccggcaccgagagacgcatccatcagtccgagttcccgaagcctgcccacgttcctgcccacagcctcccgcgccctgacaacccagccgactttcttccaactccag

SEQ ID NO: 8881 - RNA, 3117 nt, Homo sapiens
  source 1..3117: mol_type = other RNA
acactgtccccttctccccagggctgtatgggagcacaggcacaggggtaggtagagcttctggtcagcgaggggtagagcccacagagagaccagagagtggaccgcagtttcatgaaagcagagttatagctgccacttgtgcctgtgggcagagcaggtggtagaggggcctccaggaaagggccggggacacgggtgtccagcactaagcacagcgcactcagccgcagcctctgtctgtctccccacccgcccacctctggcacacagcacctggggacccagatttgtgcttgatcagagcttcgaaggaaggcagtggcagaggcgctgggaggctgtcctggaagtggccaattctggtgtcctctgcaaagtacccctcgtccctggacaaccagaacgtgccctgacctcttccctggcccgtccccacccgcggtgtgtgatccttagacgtgagtctgcatccgccgctgcaggggtcgactggggtcagagttctgggacgaggactgggagtggtgggaggaggaagcagaagccttgctggccttgtcgaactgcacatagccatcctgcttgccgctgctgctgacgctgctgtcacactgcgtgtccaggaaggagctgctgtcgctgagggagcctctctggaactcccgctcacaaagctcgatggacgagctgcccatgcccagcacaaaccgctgcccgtagtcgtagaggcggccctggccgctcagggtgctgtagatgttggtgaaggacatgcctgtgggcacacgctgcttgcccgcaggacgcaggtcgggctggcagctggagagggagatggtcggggttgagtggtgctctttgaaggtgttgacgctgtagtagccattggtggggtccttcaggttctgaaactctttctcctcttctttgaggacctccagctgtttcaggactgagtcttgctggaattcaccccggtccatcatcagctgcttgatggtggagtgctcctcaccctcccgaccagaggctggttccttgtggacaatttccactcggatatcatttttggctgacacaacacctttgagatttctctgggaacgggcacagcagaacgccacgatggttgccataaggacgaggaaggccacaccagctcctacggccaccccaatgatgacggccatcggcacagactcttgctccttgagccggatgatctcagtgtcggagccgaagctgttccaggccgtgcagttgtagatggtctggaagtcggcccgcacgatgttgctgatggtcagggtggagatgacgccctcctcggtgctgatggtctccaccgtatagcgccccgatgtgcccgactccagaacgttctccttccaggaccaggcgatgcggtccggcggcggcgtgctccggatgaagcacttgatctggcccttctcgccgtggagggcgtgctgggtctgggtgctggagatgatggggggtccattgacggtcagggtcacctctctctccccggctcccacacggggcaccacagcccggcacacgtacttgcccgcgtcctcctggcgcacggatttgagggtcagggtcttctcattgctcaggaccactccggagccccgcttcatccagacgatggtcagggatgggttgccggtccaggcgcagctgaagatggcatcagagcccagatccacgagcaaggattggggttctgtggtcatccggggcccaaagtagacgtcaaccgtgcggctgaggttggtgctgcccagggcgttggtcacctcacaggagacgggctctgagaagtacgtgtagtccactgtggtcctgtacacctctccagatgcctccttgatgatctggccccgcttggcccacctgtactgggtgacagctgggttggcctttgcagagcagtggaaagtgacgacgttgtcctccagcactggctgtggctccaccgagaggttgaccagtggagggtgctggatgtcaatggtgaccgacgtctcctttcctccggggatggctttgttggtggcacgacacacgatgctctggccattctccacgtcaccaggggagatgaagagggtgctgacgatgctctcccgcttgccgtcccgaagcagggtcttggagtaggtggccccattgatgacctctccctttcgcaaccagatgatggaggctgcaggcttggcattgtctgcgtggcaggtgaggttgagagggtcccccgcacgcaggctgatcacagggccccccaggatgacggggtcatcaggcggcaccaggactgtgaggcgtgcggggcgggagcggatggcggcctggatggcctggcactcgtacaccgcatcgtcttgcagctctgccctcaggatcttcaggtggtgctcccctgacaggtggttccctaccaccaggtactgtgggtaacttgagaggtccctgcccacacccagagccaagccgtccttgatccacagaacgaagccatcgtattcggggatggcgcaaagtagcgtcactggctgtcccgacaccaccacctggtcctggggctgctggctgaaggaatagacttggccttcattcattctccgaaacttgtccttggccatgtagcccagcaccagacagcatcctctcttctggaggcccagctcttgactgaagaggaagaagcagacgaagagcagatcgagctggaagggtttcattccttagcgcagcgaaggaaagccggcggggtaacttggctgtggttagtttctcttccttggcggctctcggtgctcagcctccgccggtcctctcgggttcgcgcctaccatctgtccgtccgtgggtccctccgggtggcttcggtctctttgtgcctctgggtatctgcagccagccgacacaaactgcctgttcttagccgcctcgggaagccgggattgtcagcaatgtccccactcggagaagatccattctctggctcttggcatcccaggcacacggcttcctcaggcgggctcctcccacagtgagcgagcgagctagtgacgagtgacagaaggactcctttcactgaag

SEQ ID NO: 8882 - RNA, 3322 nt, Homo sapiens
  source 1..3322: mol_type = other RNA
acactgtccccttctccccagggctgtatgggagcacaggcacaggggtaggtagagcttctggtcagcgaggggtagagcccacagagagaccagagagtggaccgcagtttcatgaaagcagagttatagctgccacttgtgcctgtgggcagagcaggtggtagaggggcctccaggaaagggccggggacacgggtgtccagcactaagcacagcgcactcagccgcagcctctgtctgtctccccacccgcccacctctggcacacagcacctggggacccagatttgtgcttgatcagagcttcgaaggaaggcagtggcagaggcgctgggaggctgtcctggaagtggccaattctggtgtcctctgcaaagtacccctcgtccctggacaaccagaacgtgccctgacctcttccctggcccgtccccacccgcggtgtgtgatccttagacgtgagtctgcatccgccgctgcaggggtcgactggggtcagagttctgggacgaggactgggagtggtgggaggaggaagcagaagccttgctggccttgtcgaactgcacatagccatcctgcttgccgctgctgctgacgctgctgtcacactgcgtgtccaggaaggagctgctgtcgctgagggagcctctctggaactcccgctcacaaagctcgatggacgagctgcccatgcccagcacaaaccgctgcccgtagtcgtagaggcggccctggccgctcagggtgctgtagatgttggtgaaggacatgcctgtgggcacacgctgcttgcccgcaggacgcaggtcgggctggcagctggagagggagatggtcggggttgagtggtgctctttgaaggtgttgacgctgtagtagccattggtggggtccttcaggttctgaaactctttctcctcttctttgaggacctccagctgtttcaggactgagtcttgctggaattcaccccggtccatcatcagctgcttgatggtggagtgctcctcaccctcccgaccagaggctggttccttgtggacaatttccactcggatatcatttttggctgacacaacacctttgagatttctctgggaacgggcacagcagaacgccacgatggttgccataaggacgaggaaggccacaccagctcctacggccaccccaatgatgacggccatcggcacagactcttgctccttgagccggatgatctcagtgtcggagccgaagctgttccaggccgtgcagttgtagatggtctggaagtcggcccgcacgatgttgctgatggtcagggtggagatgacgccctcctcggtgctgatggtctccaccgtatagcgccccgatgtgcccgactccagaacgttctccttccaggaccaggcgatgcggtccggcggcggcgtgctccggatgaagcacttgatctggcccttctcgccgtggagggcgtgctgggtctgggtgctggagatgatggggggtccattgacggtcagggtcacctctctctccccggctcccacacggggcaccacagcccggcacacgtacttgcccgcgtcctcctggcgcacggatttgagggtcagggtcttctcattgctcaggaccactccggagccccgcttcatccagacgatggtcagggatgggttgccggtccaggcgcagctgaagatggcatcagagcccagatccacgagcaaggattggggttctgtggtcatccggggcccaaagtagacgtcaaccgtgcggctgaggttggtgctgcccagggcgttggtcacctcacaggagacgggctctgagaagtacgtgtagtccactgtggtcctgtacacctctccagatgcctccttgatgatctggccccgcttggcccacctgtactgggtgacagctgggttggcctttgcagagcagtggaaagtgacgacgttgtcctccagcactggctgtggctccaccgagaggttgaccagtggagggtgctggatgtcaatggtgaccgacgtctcctttcctccggggatggctttgttggtggcacgacacacgatgctctggccattctccacgtcaccaggggagatgaagagggtgctgacgatgctctcccgcttgccgtcccgaagcagggtcttggagtaggtggccccattgatgacctctccctttcgcaaccagatgatggaggctgcaggcttggcattgtctgcgtggcaggtgaggttgagagggtcccccgcacgcaggctgatcacagggccccccaggatgacggggtcatcaggcggcaccaggactgtgaggcgtgcggggcgggagcggatggcggcctggatggcctggcactcgtacaccgcatcgtcttgcagctctgccctcaggatcttcaggtggtgctcccctgacaggtggttccctaccaccaggtactgtgggtaacttgagaggtccctgcccacacccagagccaagccgtccttgatccacagaacgaagccatcgtattcggggatggcgcaaagtagcgtcactggctgtcccgacaccaccacctggtcctggggctgctggctgaaggaatagacttggccttcattcattctccgaaacttgtccttggccatgtagcccagcaccagacagcatcctctcttctggaggcccagctcttgactgaagaggaagaagcagacgaagagcagatcgagctggaagggtttcattccttagcgcagcgaaggaaagccggcggggtaacttggctgtggttagtttctcttccttggcggctctcggtgctcagcctccgccggtcctctcgggttcgcgcctaccatctgtccgtccgtgggtccctccgggtggcttcggtctctttgtgcctctgggtatctgcagccagccgacacaaactgcctgttcttagccgcctcgggaagccgggattgtcagcaatgtccccactcggagaagatccattctctggctcttggcatcccaggcacacggcttcctcaggcgggctcctcccacagtgagcgagcgagctagtgacgagtgacagaaggactcctttcactgaagctgcaggacccacagccggtcgggctctggcgccagcctcgacggcggccccgccatctccgcccggctgcccgcggcctcacctcctccgggggctcggttagcctcctggcgctgcaaggctgcctgcgcgcggttcgctccgggggagggaggaggagggaggcggcgaggagccgacggctccacctgatggagaagcgcg

SEQ ID NO: 8883 - RNA, 2972 nt, Homo sapiens
  source 1..2972: mol_type = other RNA
acactgtccccttctccccagggctgtatgggagcacaggcacaggggtaggtagagcttctggtcagcgaggggtagagcccacagagagaccagagagtggaccgcagtttcatgaaagcagagttatagctgccacttgtgcctgtgggcagagcaggtggtagaggggcctccaggaaagggccggggacacgggtgtccagcactaagcacagcgcactcagccgcagcctctgtctgtctccccacccgcccacctctggcacacagcacctggggacccagatttgtgcttgatcagagcttcgaaggaaggcagtggcagaggcgctgggaggctgtcctggaagtggccaattctggtgtcctctgcaaagtacccctcgtccctggacaaccagaacgtgccctgacctcttccctggcccgtccccacccgcggtgtgtgatccttagacgtgagtctgcatccgccgctgcaggggtcgactggggtcagagttctgggacgaggactgggagtggtgggaggaggaagcagaagccttgctggccttgtcgaactgcacatagccatcctgcttgccgctgctgctgacgctgctgtcacactgcgtgtccaggaaggagctgctgtcgctgagggagcctctctggaactcccgctcacaaagctcgatggacgagctgcccatgcccagcacaaaccgctgcccgtagtcgtagaggcggccctggccgctcagggtgctgtagatgttggtgaaggacatgcctgtgggcacacgctgcttgcccgcaggacgcaggtcgggctggcagctggagagggagatggtcggggttgagtggtgctctttgaaggtgttgacgctgtagtagccattggtggggtccttcaggttctgaaactctttctcctcttctttgaggacctccagctgtttcaggactgagtcttgctggaattcaccccggtccatcatcagctgcttgatggtggagtgctcctcaccctcccgaccagaggctggttccttgtggacaatttccactcggatatcatttttggctgacacaacacctttgagatttgctctccggggcagcctaagcctggcctttttctctgtccccctccctgagatcccggatctccctcccgtacttctctgggaacgggcacagcagaacgccacgatggttgccataaggacgaggaaggccacaccagctcctacggccaccccaatgatgacggccatcggcacagactctgcttccagcccggctcccgacttcatttccgaaccttgctccttgagccggatgatctcagtgtcggagccgaagctgttccaggccgtgcagttgtagatggtctggaagtcggcccgcacgatgttgctgatggtcagggtggagatgacgccctcctcggtgctgatggtctccaccgtatagcgccccgatgtgcccgactccagaacgttctccttccaggaccaggcgatgcggtccggcggcggcgtgctccggatgaagcacttgatctggcccttctcgccgtggagggcgtgctgggtctgggtgctggagatgatggggggtccattgacggtcagggtcacctctctctccccggctcccacacggggcaccacagcccggcacacgtacttgcccgcgtcctcctggcgcacggatttgagggtcagggtcttctcattgctcaggaccactccggagccccgcttcatccagacgatggtcagggatgggttgccggtccaggcgcagctgaagatggcatcagagcccagatccacgagcaaggattggggttctgtggtcatccggggcccaaagtagacgtcaaccgtgcggctgaggttggtgctgcccagggcgttggtcacctcacaggagacgggctctgagaagtacgtgtagtccactgtggtcctgtacacctctccagatgcctccttgatgatctggccccgcttggcccacctgtactgggtgacagctgggttggcctttgcagagcagtggaaagtgacgacgttgtcctccagcactggctgtggctccaccgagaggttgaccagtggagggtgctggatgtcaatggtgaccgacgtctcctttcctccggggatggctttgttggtggcacgacacacgatgctctggccattctccacgtcaccaggggagatgaagagggtgctgacgatgctctcccgcttgccgtcccgaagcagggtcttggagtaggtggccccattgatgacctctccctttcgcaaccagatgatggaggctgcaggcttggcattgtctgcgtggcaggtgaggttgagagggtcccccgcacgcaggctgatcacagggccccccaggatgacggggtcatcaggcggcaccaggactgtgaggcgtgcggggcgggagcggatggcggcctggatggcctggcactcgtacaccgcatcgtcttgcagctctgccctcaggatcttcaggtggtgctcccctgacaggtggttccctaccaccaggtactgtgggtaacttgagaggtccctgcccacacccagagccaagccgtccttgatccacagaacgaagccatcgtattcggggatggcgcaaagtagcgtcactggctgtcccgacaccaccacctggtcctggggctgctggctgaaggaatagacttggccttcattcattctccgaaacttgtccttggccatgtagcccagcaccagacagcatcctctcttctggaggcccagctcattttgttgcattcgcaaaggcgaagaggcaatgccagagcatctcagcccggcaccgagagacgcatccatcagtccgagttcccgaagcctgcccacgttcctgcccacagcctcccgcgccctgacaacccagccgactttcttccaactccagca

SEQ ID NO: 8884 - RNA, 3292 nt, Homo sapiens
  source 1..3292: mol_type = other RNA
acactgtccccttctccccagggctgtatgggagcacaggcacaggggtaggtagagcttctggtcagcgaggggtagagcccacagagagaccagagagtggaccgcagtttcatgaaagcagagttatagctgccacttgtgcctgtgggcagagcaggtggtagaggggcctccaggaaagggccggggacacgggtgtccagcactaagcacagcgcactcagccgcagcctctgtctgtctccccacccgcccacctctggcacacagcacctggggacccagatttgtgcttgatcagagcttcgaaggaaggcagtggcagaggcgctgggaggctgtcctggaagtggccaattctggtgtcctctgcaaagtacccctcgtccctggacaaccagaacgtgccctgacctcttccctggcccgtccccacccgcggtgtgtgatccttagacgtgagtctgcatccgccgctgcaggggtcgactggggtcagagttctgggacgaggactgggagtggtgggaggaggaagcagaagccttgctggccttgtcgaactgcacatagccatcctgcttgccgctgctgctgacgctgctgtcacactgcgtgtccaggaaggagctgctgtcgctgagggagcctctctggaactcccgctcacaaagctcgatggacgagctgcccatgcccagcacaaaccgctgcccgtagtcgtagaggcggccctggccgctcagggtgctgtagatgttggtgaaggacatgcctgtgggcacacgctgcttgcccgcaggacgcaggtcgggctggcagctggagagggagatggtcggggttgagtggtgctctttgaaggtgttgacgctgtagtagccattggtggggtccttcaggttctgaaactctttctcctcttctttgaggacctccagctgtttcaggactgagtcttgctggaattcaccccggtccatcatcagctgcttgatggtggagtgctcctcaccctcccgaccagaggctggttccttgtggacaatttccactcggatatcatttttggctgacacaacacctttgagatttgctctccggggcagcctaagcctggcctttttctctgtccccctccctgagatcccggatctccctcccgtacttctctgggaacgggcacagcagaacgccacgatggttgccataaggacgaggaaggccacaccagctcctacggccaccccaatgatgacggccatcggcacagactctgcttccagcccggctcccgacttcatttccgaaccttgctccttgagccggatgatctcagtgtcggagccgaagctgttccaggccgtgcagttgtagatggtctggaagtcggcccgcacgatgttgctgatggtcagggtggagatgacgccctcctcggtgctgatggtctccaccgtatagcgccccgatgtgcccgactccagaacgttctccttccaggaccaggcgatgcggtccggcggcggcgtgctccggatgaagcacttgatctggcccttctcgccgtggagggcgtgctgggtctgggtgctggagatgatggggggtccattgacggtcagggtcacctctctctccccggctcccacacggggcaccacagcccggcacacgtacttgcccgcgtcctcctggcgcacggatttgagggtcagggtcttctcattgctcaggaccactccggagccccgcttcatccagacgatggtcagggatgggttgccggtccaggcgcagctgaagatggcatcagagcccagatccacgagcaaggattggggttctgtggtcatccggggcccaaagtagacgtcaaccgtgcggctgaggttggtgctgcccagggcgttggtcacctcacaggagacgggctctgagaagtacgtgtagtccactgtggtcctgtacacctctccagatgcctccttgatgatctggccccgcttggcccacctgtactgggtgacagctgggttggcctttgcagagcagtggaaagtgacgacgttgtcctccagcactggctgtggctccaccgagaggttgaccagtggagggtgctggatgtcaatggtgaccgacgtctcctttcctccggggatggctttgttggtggcacgacacacgatgctctggccattctccacgtcaccaggggagatgaagagggtgctgacgatgctctcccgcttgccgtcccgaagcagggtcttggagtaggtggccccattgatgacctctccctttcgcaaccagatgatggaggctgcaggcttggcattgtctgcgtggcaggtgaggttgagagggtcccccgcacgcaggctgatcacagggccccccaggatgacggggtcatcaggcggcaccaggactgtgaggcgtgcggggcgggagcggatggcggcctggatggcctggcactcgtacaccgcatcgtcttgcagctctgccctcaggatcttcaggtggtgctcccctgacaggtggttccctaccaccaggtactgtgggtaacttgagaggtccctgcccacacccagagccaagccgtccttgatccacagaacgaagccatcgtattcggggatggcgcaaagtagcgtcactggctgtcccgacaccaccacctggtcctggggctgctggctgaaggaatagacttggccttcattcattctccgaaacttgtccttggccatgtagcccagcaccagacagcatcctctcttctggaggcccagctcttgactgaagaggaagaagcagacgaagagcagatcgagctggaagggtttcattccttagcgcagcgaaggaaagccggcggggtaacttggctgtggttagtttctcttccttggcggctctcggtgctcagcctccgccggtcctctcgggttcgcgcctaccatctgtccgtccgtgggtccctccgggtggcttcggtctctttgtgcctctgggtatctgcagccagccgacacaaactgcctgttcttagccgcctcgggaagccgggattgtcagcaatgtccccactcggagaagatccattctctggctcttggcatcccaggcacacggcttcctcaggcgggctcctcccacagtgagcgagcgagctagtgacgagtgacagaaggactcctttcactgaagctcctccgggggctcggttagcctcctggcgctgcaaggctgcctgcgcgcggttcgctccggg

SEQ ID NO: 8885 - RNA, 3433 nt, Homo sapiens
  source 1..3433: mol_type = other RNA
acactgtccccttctccccagggctgtatgggagcacaggcacaggggtaggtagagcttctggtcagcgaggggtagagcccacagagagaccagagagtggaccgcagtttcatgaaagcagagttatagctgccacttgtgcctgtgggcagagcaggtggtagaggggcctccaggaaagggccggggacacgggtgtccagcactaagcacagcgcactcagccgcagcctctgtctgtctccccacccgcccacctctggcacacagcacctggggacccagatttgtgcttgatcagagcttcgaaggaaggcagtggcagaggcgctgggaggctgtcctggaagtggccaattctggtgtcctctgcaaagtacccctcgtccctggacaaccagaacgtgccctgacctcttccctggcccgtccccacccgcggtgtgtgatccttagacgtgagtctgcatccgccgctgcaggggtcgactggggtcagagttctgggacgaggactgggagtggtgggaggaggaagcagaagccttgctggccttgtcgaactgcacatagccatcctgcttgccgctgctgctgacgctgctgtcacactgcgtgtccaggaaggagctgctgtcgctgagggagcctctctggaactcccgctcacaaagctcgatggacgagctgcccatgcccagcacaaaccgctgcccgtagtcgtagaggcggccctggccgctcagggtgctgtagatgttggtgaaggacatgcctgtgggcacacgctgcttgcccgcaggacgcaggtcgggctggcagctggagagggagatggtcggggttgagtggtgctctttgaaggtgttgacgctgtagtagccattggtggggtccttcaggttctgaaactctttctcctcttctttgaggacctccagctgtttcaggactgagtcttgctggaattcaccccggtccatcatcagctgcttgatggtggagtgctcctcaccctcccgaccagaggctggttccttgtggacaatttccactcggatatcatttttggctgacacaacacctttgagatttgctctccggggcagcctaagcctggcctttttctctgtccccctccctgagatcccggatctccctcccgtacttctctgggaacgggcacagcagaacgccacgatggttgccataaggacgaggaaggccacaccagctcctacggccaccccaatgatgacggccatcggcacagactctgcttccagcccggctcccgacttcatttccgaaccttgctccttgagccggatgatctcagtgtcggagccgaagctgttccaggccgtgcagttgtagatggtctggaagtcggcccgcacgatgttgctgatggtcagggtggagatgacgccctcctcggtgctgatggtctccaccgtatagcgccccgatgtgcccgactccagaacgttctccttccaggaccaggcgatgcggtccggcggcggcgtgctccggatgaagcacttgatctggcccttctcgccgtggagggcgtgctgggtctgggtgctggagatgatggggggtccattgacggtcagggtcacctctctctccccggctcccacacggggcaccacagcccggcacacgtacttgcccgcgtcctcctggcgcacggatttgagggtcagggtcttctcattgctcaggaccactccggagccccgcttcatccagacgatggtcagggatgggttgccggtccaggcgcagctgaagatggcatcagagcccagatccacgagcaaggattggggttctgtggtcatccggggcccaaagtagacgtcaaccgtgcggctgaggttggtgctgcccagggcgttggtcacctcacaggagacgggctctgagaagtacgtgtagtccactgtggtcctgtacacctctccagatgcctccttgatgatctggccccgcttggcccacctgtactgggtgacagctgggttggcctttgcagagcagtggaaagtgacgacgttgtcctccagcactggctgtggctccaccgagaggttgaccagtggagggtgctggatgtcaatggtgaccgacgtctcctttcctccggggatggctttgttggtggcacgacacacgatgctctggccattctccacgtcaccaggggagatgaagagggtgctgacgatgctctcccgcttgccgtcccgaagcagggtcttggagtaggtggccccattgatgacctctccctttcgcaaccagatgatggaggctgcaggcttggcattgtctgcgtggcaggtgaggttgagagggtcccccgcacgcaggctgatcacagggccccccaggatgacggggtcatcaggcggcaccaggactgtgaggcgtgcggggcgggagcggatggcggcctggatggcctggcactcgtacaccgcatcgtcttgcagctctgccctcaggatcttcaggtggtgctcccctgacaggtggttccctaccaccaggtactgtgggtaacttgagaggtccctgcccacacccagagccaagccgtccttgatccacagaacgaagccatcgtattcggggatggcgcaaagtagcgtcactggctgtcccgacaccaccacctggtcctggggctgctggctgaaggaatagacttggccttcattcattctccgaaacttgtccttggccatgtagcccagcaccagacagcatcctctcttctggaggcccagctcttgactgaagaggaagaagcagacgaagagcagatcgagctggaagggtttcattccttagcgcagcgaaggaaagccggcggggtaacttggctgtggttagtttctcttccttggcggctctcggtgctcagcctccgccggtcctctcgggttcgcgcctaccatctgtccgtccgtgggtccctccgggtggcttcggtctctttgtgcctctgggtatctgcagccagccgacacaaactgcctgttcttagccgcctcgggaagccgggattgtcagcaatgtccccactcggagaagatccattctctggctcttggcatcccaggcacacggcttcctcaggcgggctcctcccacagtgagcgagcgagctagtgacgagtgacagaaggactcctttcactgaagctgcaggacccacagccggtcgggctctggcgccagcctcgacggcggccccgccatctccgcccggctgcccgcggcctcacctcctccgggggctcggttagcctcctggcgctgcaaggctgcctgcgcgcggttcgctccgggggagggaggaggagggaggcggcgaggagccgacggctccacctgatggagaagcgcg

SEQ ID NO: 8886 - RNA, 3397 nt, Homo sapiens
  source 1..3397: mol_type = other RNA
acactgtccccttctccccagggctgtatgggagcacaggcacaggggtaggtagagcttctggtcagcgaggggtagagcccacagagagaccagagagtggaccgcagtttcatgaaagcagagttatagctgccacttgtgcctgtgggcagagcaggtggtagaggggcctccaggaaagggccggggacacgggtgtccagcactaagcacagcgcactcagccgcagcctctgtctgtctccccacccgcccacctctggcacacagcacctggggacccagatttgtgcttgatcagagcttcgaaggaaggcagtggcagaggcgctgggaggctgtcctggaagtggccaattctggtgtcctctgcaaagtacccctcgtccctggacaaccagaacgtgccctgacctcttccctggcccgtccccacccgcggtgtgtgatccttagacgtgagtctgcatccgccgctgcaggggtcgactggggtcagagttctgggacgaggactgggagtggtgggaggaggaagcagaagccttgctggccttgtcgaactgcacatagccatcctgcttgccgctgctgctgacgctgctgtcacactgcgtgtccaggaaggagctgctgtcgctgagggagcctctctggaactcccgctcacaaagctcgatggacgagctgcccatgcccagcacaaaccgctgcccgtagtcgtagaggcggccctggccgctcagggtgctgtagatgttggtgaaggacatgcctgtgggcacacgctgcttgcccgcaggacgcaggtcgggctggcagctggagagggagatggtcggggttgagtggtgctctttgaaggtgttgacgctgtagtagccattggtggggtccttcaggttctgaaactctttctcctcttctttgaggacctccagctgtttcaggactgagtcttgctggaattcaccccggtccatcatcagctgcttgatggtggagtgctcctcaccctcccgaccagaggctggttccttgtggacaatttccactcggatatcatttttggctgacacaacacctttgagatttgctctccggggcagcctaagcctggcctttttctctgtccccctccctgagatcccggatctccctcccgtacttctctgggaacgggcacagcagaacgccacgatggttgccataaggacgaggaaggccacaccagctcctacggccaccccaatgatgacggccatcggcacagactcttgctccttgagccggatgatctcagtgtcggagccgaagctgttccaggccgtgcagttgtagatggtctggaagtcggcccgcacgatgttgctgatggtcagggtggagatgacgccctcctcggtgctgatggtctccaccgtatagcgccccgatgtgcccgactccagaacgttctccttccaggaccaggcgatgcggtccggcggcggcgtgctccggatgaagcacttgatctggcccttctcgccgtggagggcgtgctgggtctgggtgctggagatgatggggggtccattgacggtcagggtcacctctctctccccggctcccacacggggcaccacagcccggcacacgtacttgcccgcgtcctcctggcgcacggatttgagggtcagggtcttctcattgctcaggaccactccggagccccgcttcatccagacgatggtcagggatgggttgccggtccaggcgcagctgaagatggcatcagagcccagatccacgagcaaggattggggttctgtggtcatccggggcccaaagtagacgtcaaccgtgcggctgaggttggtgctgcccagggcgttggtcacctcacaggagacgggctctgagaagtacgtgtagtccactgtggtcctgtacacctctccagatgcctccttgatgatctggccccgcttggcccacctgtactgggtgacagctgggttggcctttgcagagcagtggaaagtgacgacgttgtcctccagcactggctgtggctccaccgagaggttgaccagtggagggtgctggatgtcaatggtgaccgacgtctcctttcctccggggatggctttgttggtggcacgacacacgatgctctggccattctccacgtcaccaggggagatgaagagggtgctgacgatgctctcccgcttgccgtcccgaagcagggtcttggagtaggtggccccattgatgacctctccctttcgcaaccagatgatggaggctgcaggcttggcattgtctgcgtggcaggtgaggttgagagggtcccccgcacgcaggctgatcacagggccccccaggatgacggggtcatcaggcggcaccaggactgtgaggcgtgcggggcgggagcggatggcggcctggatggcctggcactcgtacaccgcatcgtcttgcagctctgccctcaggatcttcaggtggtgctcccctgacaggtggttccctaccaccaggtactgtgggtaacttgagaggtccctgcccacacccagagccaagccgtccttgatccacagaacgaagccatcgtattcggggatggcgcaaagtagcgtcactggctgtcccgacaccaccacctggtcctggggctgctggctgaaggaatagacttggccttcattcattctccgaaacttgtccttggccatgtagcccagcaccagacagcatcctctcttctggaggcccagctcttgactgaagaggaagaagcagacgaagagcagatcgagctggaagggtttcattccttagcgcagcgaaggaaagccggcggggtaacttggctgtggttagtttctcttccttggcggctctcggtgctcagcctccgccggtcctctcgggttcgcgcctaccatctgtccgtccgtgggtccctccgggtggcttcggtctctttgtgcctctgggtatctgcagccagccgacacaaactgcctgttcttagccgcctcgggaagccgggattgtcagcaatgtccccactcggagaagatccattctctggctcttggcatcccaggcacacggcttcctcaggcgggctcctcccacagtgagcgagcgagctagtgacgagtgacagaaggactcctttcactgaagctgcaggacccacagccggtcgggctctggcgccagcctcgacggcggccccgccatctccgcccggctgcccgcggcctcacctcctccgggggctcggttagcctcctggcgctgcaaggctgcctgcgcgcggttcgctccgggggagggaggaggagggaggcggcgaggagccgacggctccacctgatggagaagcgcg

SEQ ID NO: 8887 - RNA, 88 nt, Homo sapiens
  source 1..88: mol_type = other RNA
acagacttgctgtgatgttcacgtggagaggagttaaacatcactgcaagtcttaacagccgcccgcccaaggcacaggggacagggc

SEQ ID NO: 8888 - RNA, 8805 nt, Homo sapiens
  source 1..8805: mol_type = other RNA
acagcactgcctggtcagaaattctcaaatgcttttgttctgtgagacatacagaataaataccattactatatcttacatcttgccttccctgaccactcagaactggggctggagcaccagccaaggcagacaaacaaggtttccttagttggccataaagcagtgataatcaactttggctggacattagaaccgccttggaggctttcgcaaatattggtgtctggttcccactccaaatgattttaatataattgggaatttaaaaatttcctgaggtgattcttatgtacagtcaaggttgagaatcactcctctagataaatgtgtaaatcaaagcatccatctgtgcatctgattccttaaagcctctttcacttcactgtggctcccatgtccttcctcaccacgatcttcttgcaccaaattggtacttcctcctccttttctaagacagaccttacctattctacatttcatgctttcagggctatgttgtctgcaaatacacacactaaacttgttatgttgacaaccatgttccctggaatggtgcatactagaggtactgctcaaaccaagtacaccacaagtatttctggcacccaggacagtgtgcatgtgaaatagtacctagccaaaaatggagttgcatgacagaggacagaggtgaagaagctgtgaaagccaccacgtttctcctgacacagataccaagacctgatatgaatgttttgacttcttttgcattgccctgtgtgagccaacatggtcaagttacaattcttttttctcatagcagcaggttgtaatcacacagatatactcccagtttgacccaatgatcctaagccaaggagaggatttttagcttacttttctagattggcttcatttttcccttctgcttgaatataagaatctattttaatcttcttcaaccaatgttaggcctaatctgattcttttttctctcaaagtcatggtgatcccttcatgtagataaagtatagatgatgcctttaaaactggtacatgggtcacataaaaagggactccaacagtaaaccttttccttcagatccctagaaactttgagggaaaggagttggattttgatttatttatttgagaatcactttcaaaagatctgagaaaattgtctttgtgactgaatcactggaaaacatctcattcagttctgtcactgtcctttcagagttccagttagacaatgatcttgacaatgattggggccctaaagtctggggctcagtgaagtgtaagaagcaaagtcagtagtactgcttttgtaggtgattaaaacaaatgaggaatcaatcattcctccctccaaactccaagactaatggatgatttcaaggtagggactattgctcacgttattatcagggaaacaaatacctctagcttctcacagatgaataaatgaaaaggcccattttctactgtaacactaaaaaggccttatcttccaaggaaatcatagggagacaaggtcaacttgttgggactgtggtttgcaagccttatcttctgatgtcgctttagcagatagaatgtaattttgatggtaactaaggctcagagtcactttctgtatcattgtccaagttattaggagtatttttcttatgttccgaaatagaagaaagatagtaaagatgagactatgcaaaggattacatggatcaacagtacttattttccaaagatgaggataagatgatgatggtagtggtggcgatggtgtgtgtgtgtgtgcgtgcgtgctaaggtcagtgcaacagaacagaattgttcaaagagaaaaatcacatccacattagattcttcttattgctatcatctctttgaattataaaaataattttgatacagtaaaacctcattaatttggattccactaaccaggagtttgtgagatgaagttacccttacgttaaggaagggcttataaaagcaattttgaaagacacgttttaactacttcaaagagccttttcttttcaagcatttgagaagcacctgtttacttccaattggtgtgctaattataaacttttgatctattcactgaggccaaggttttaagcacttctacagtgaaatgctataatgtcctttttgatattttctctgtgtgccttaaaatattctgtagttgttatttttcactgattcctataagctttcttcaaaattgtatcttattgcatatgaaccacacatgtaattttgggtataataatttatcttgctaagacattgtatacttattgtacagttttatacaacaacatatattacatattcacacaatctacctctttgtatgatgtagaatagtggctgtgaactgggagaaattttggcaatgactggagacattttgattgtcattactaggaggttcttactggcatctagtagacagaggccagggatgttgctaacatcctacaatacacaggacagttccccacaacaaagactttcagctaatagtgctgcttttgagaaatctcgatgtagatcaagttaaaacaagttaaatcttattgaaggcttcagaaatactcatcaaatgtactgctactttggactgaatttcattatttctaaaataaactaatattttactcttttagttttttttaaaatacagaaacgataaagtatttgttctgaaaatcagaaaactaagtctttgaaacagatggtacaaagaatacattgcaatttggccactagtattttctagatcctactcttaagtttctttaatatttttaccatataattttataattctataaattatacagtcatgtaatgtctgtgtttccaagccagattctgttaccgtaaggctgttcacaggagtctgggagattcagagaggctttcttaacaagaggattcaaggactctgagaaatgctatcctagtgtacattatctaactctttcactcatctttgttctcctcaaaattactgagaacattgtaccactagaaacatttgctagaaagtacaacttctagcaaaaaattagactaaaaaggaaataaaaatacgattttttggctaataaaataacctgaaatccaggaaaattgtgaagtcttaagaaacacaaatgtaaatccaatgagaccttgataaacaaaaattcaataagccaaaaccataattaaaacttttcttgacgaaacaacatattacaggatgggtcctggaatgtgtatatatacattcctataacttttgacttccagaatcatgttaaatggtagtaggtgtctctatttggttttgactctggtgcttttctggtgagttatagataccttgtatcatgttaaggatattctttattccagctttaaaagagtctttaataagggacaagtgtttggcatctattgacataatctagtggcttatattatttgacctagggacaaaagcattgattttgtatcattaaactctttatgtatttctattgtctataatgatgactgagaccaagatagcaaacagatcactatattttataaagatttccagtggtaagtatcgaaccaatttccagtggtaagtatcaaaccgaaaggtattttctaaggaaagcccttgtaaatcagaaatgtcataaatcagaatccctttcccaaaacattaactgagattttactgaatcacactaaagagaatgaccagtttggtttgtgaatgtcaggctgcaagagcacctttcgattgcagaccctactgggtttgaacagtaatatactgtgtaactggcagacaaggatacaaatgaagcttttaaaatatatcactttagaagctgaaattggggtgtgtgaaatttccctttttgtgaagtcagttctcatagctaactctattgttcctatagattccccacacctactaccaactcccctatagagtacaagccaggctgaagaaaatgctttgaggtgacccaaccctgcatggtttgtgctaaaaacagcaacccattctgaaggtgatagaaatgaaactgattgtgttgggaataatttactatactggcaatatttgattttgacacaactgtgaatgatgtaaaacatggagagagaacattaatcagactcttgccataagaattcaataaggttctagtacaatgaaagttacagatgaggagaaaactctgggttcttgttttgttttgttttccgtttcagttgggtatggcaaatatatttgaaatgcactgacatcttcaaatgcagattttttaaattgttgagtgtggcccaattgatagaaatagtttaccatgaatctttttttcttctatcacaacatgcttttttttcttttccccttaagatgttaatttatcatgcaaagattttttttcattaagtgcattaatgcttttgtttgtacaggaattttcaaatcaagaggactccccgtagttactaaatataaatccttatcgaatgacatgccaagatgatagctccattccacatgggaaaaggcaaattcagccgtattttgggattttaaccagggctccagcctttgggttgcacagtgtctctgatacatctcttttatgaaaatttcagattgactgtaaatggaacattttgtagaagaaactggcttctagcagttgagtagtgatgctgggaataaatttggtttccctgaatatggtttctcaaagcagtcacagcttctttagaagtcagaattggtaccatttcttatccttgtatttcagcattaactcatgtgcatgtttggaaaatgcttctgcactggtcatcatgcctgcagttttctcttccagctctcctagcctctgtcctctttcatcaagtgcaatccgtgcacgggtcagctctcccatcacccctccagcagcgcctttcatcccttctatactacctggtccaggaatgtgttgcgcaaggctgcgggatgcttttcctgccgaagcttccccaaagagctcttctctgtcaaatgtttgtccgcttccaccaaacagtcccttgagaaagcctctgttttgagcttctggtgtctctatgggagtaaacaaatctcctagcatgtcctgtagattatcacacatttcttggctgtatgttaaccgctgaatttcagtaggagagacgaggtataatgcctgtccttcattggtaaaacaaaatgttcgtgctatcctcatgtctgtcagtggcaaataattaacatccaacattgggcgaagactaggtaggctcattatcatgatatgtccgttagcacaaaagcatgccaagcaggcactgctacacatgaccaccacatttgcttgcagtataaaagatgtctccgtgatgttatgaacataaaggcaagtctgagaaggcagtgagaagactttggcttgtttttctgagcagattattgtatactgatgatctcctatttcttgggatgcagaagatgagttcattaccactttccttctccaagatttttcattttcatctatgttgtttggatccctccaaacttcatatggcggttgcattaatccacccattcggtccatacaggagaatgttagcacagctcctttcaatgagaggaatgtaccacttggcaataccatgactggctctgtaaacctttgttcatctgctaatggtaggtttaaggagatgattaacaccattcccagactggttccaacgaacagacaaggagagatggtagagtcatttttccgtgcaaaggagtccatgaagtatagtgctgtaattgcttctttagaatctttgtcaatactggagatactagagcttctagaacgattataggaattttctcggttttcttctgttgtaactggtaaagaaatctccatgcaggctgctgactgggcctttcgaaatggtggtcttccaggaccccagcgatttacttttgaaacatcggcactagaaagacgttttccagaactgcaactctgagaagttggacttgtgcagtgtccatttacatggtctgaggtaggagacttgcagcgctcaagttctaggggaactggactgtcattcagttcagttaaacctgcaatgaactgtttgttttttcgaggagaccgtggttgtcgctggtataagtcacttgatctatataggtcaatggtccccatgcttaacagtactgtcttctgtataaaatccaccacagccaacccattgcagttcccaaatgcaactattccatatgctgagcttacagcaagactagtaatctgttgtggaggttcaccatctacccacaccaattgaataacaagttctgcttgatatcctggaggcattcgcactggccgtgtcttcacattgaggcatggaatactgtcctttgttactccttcactagcaacagtgttagtgctcccagaaagactccttgaagaaggaagctgggctgagagatctggaaacggaggacttgtttctggttcaggggtaataatatcttcaacatcatactgaagtcgtacctctaatgacactatttctgttgtaatttcatgtctgctgaatttataaattatgacatatgcagagactcctgatacacagaatattctgctctctggacaccagtaaatcatctgaatggcaaatgggtcttcctctacaatttcacatgtttgttttccttctcctaccttctgtttttcaaacacttttgaagtttttagcttgtacagcatctgcagagttattgcagaagcatcccaaaattttattgatccatctgcatgaccagtaataataatttctggatatgtttgtgctccaaggttccaagctcctccactgattggccactccttattactgtatccttgttttttatgcttgactcctatagaatacagtactagaatcaaatccggaggacaatctgcaaagtatgctgtgcatgtaactggtgattcatgaatgtccatgggatatggattttcaaagattggaaaattgctttgtgtcagatcaactacaatgagatctttctccagaagtaccacgacagcatagggttcttgaaattcatttggatagggcgtttcacataaagttagaaattcaacaataggatgatccatttcaagtactgtaattgcttttccatgcatgatggttaaacttggtcttctacaagctttgtcataggacagcccaccagagaatattatgaatggttcgctgtttttgcaggtcttgtattctactttaagaattggtttacaagattcagattttcttccttctctttgactttttccatgtggaattgtggtctggaaagggcgacttgggcttttcaggttccataaagtcaaactaccatctgaatggctgcacatgaactgtttgccctcatgatgccaatcaattgaatgaatagcctcatcataataaactctcagttctgctcttttagatttcaagtcccagaatactacagtaccattttcataacctattagcagtttgccttcatctcttgggctatcgcttaaatgtacaactggacctggatgagtcttagtggatagttcaattgccttgttccacatgataacatatccagaaagaatgaaagattcaatatttacaatatgtgtatttcctctttctgttccaacataaagccatttactctggaaaggtagatgacagtaagtaattcgttcccggttaaatttaagagaatggagtatggctggccttttttgtctaaggttccacaaatgaagtgtatcatctgaacttgcactgaccaaggcaccctcattgatcaaaaattggagctgtaggacagctgcaccactttcatgttggcaatagcaatcaacaccaggtctcccgagtattcgtatagcacctgttctcgtcccaatagccaagattttctgaactggatcaaaggctaatgctgtgggctgatgaggaaaaccatgccgaactgtcttgcaaatctggaaatactccgaagtcaaagtttcctgaatttcctctctgagaacccctgcagtccccgccggatgtacggaaccacttccagccccaccaccactgttactgccactgctgctaccactgccaggggaggaggcagttaagccatccaaaacttttcggaaattaaacttcttcattttaaacacaagactctgtctctctcttaagggcggactttccttcttcgaaacgttcggctcagagtattttattttcagaaaaacgacgttgggggagccggtatttactctgccaccaccttccgggctcttcccccatcagcttcaacgcttccttttttgtcactatgaaaggcggggaggggggtactttttctagtccccatcccccagcagcccggaccccaaaacatctgcgagtgacccacagcaacagctgccggggagggggggaggaggagaacggcgacaccgtctgtttccacttgtccctccgcctccccctcacctccccctcatctccctccccgcgtcctctttcccccctctccccatctcctgctcccctccctccacctctgcccgcagccgccgccgcgctctcccgcctgttcgcccgcccgccgtccgctctccccgctgcacggcagccgctctcgggggacgtgaagcggtggcggcgacggctgcggcccgagtc

SEQ ID NO: 8889 - RNA, 8414 nt, Homo sapiens
  source 1..8414: mol_type = other RNA
acagcactgcctggtcagaaattctcaaatgcttttgttctgtgagacatacagaataaataccattactatatcttacatcttgccttccctgaccactcagaactggggctggagcaccagccaaggcagacaaacaaggtttccttagttggccataaagcagtgataatcaactttggctggacattagaaccgccttggaggctttcgcaaatattggtgtctggttcccactccaaatgattttaatataattgggaatttaaaaatttcctgaggtgattcttatgtacagtcaaggttgagaatcactcctctagataaatgtgtaaatcaaagcatccatctgtgcatctgattccttaaagcctctttcacttcactgtggctcccatgtccttcctcaccacgatcttcttgcaccaaattggtacttcctcctccttttctaagacagaccttacctattctacatttcatgctttcagggctatgttgtctgcaaatacacacactaaacttgttatgttgacaaccatgttccctggaatggtgcatactagaggtactgctcaaaccaagtacaccacaagtatttctggcacccaggacagtgtgcatgtgaaatagtacctagccaaaaatggagttgcatgacagaggacagaggtgaagaagctgtgaaagccaccacgtttctcctgacacagataccaagacctgatatgaatgttttgacttcttttgcattgccctgtgtgagccaacatggtcaagttacaattcttttttctcatagcagcaggttgtaatcacacagatatactcccagtttgacccaatgatcctaagccaaggagaggatttttagcttacttttctagattggcttcatttttcccttctgcttgaatataagaatctattttaatcttcttcaaccaatgttaggcctaatctgattcttttttctctcaaagtcatggtgatcccttcatgtagataaagtatagatgatgcctttaaaactggtacatgggtcacataaaaagggactccaacagtaaaccttttccttcagatccctagaaactttgagggaaaggagttggattttgatttatttatttgagaatcactttcaaaagatctgagaaaattgtctttgtgactgaatcactggaaaacatctcattcagttctgtcactgtcctttcagagttccagttagacaatgatcttgacaatgattggggccctaaagtctggggctcagtgaagtgtaagaagcaaagtcagtagtactgcttttgtaggtgattaaaacaaatgaggaatcaatcattcctccctccaaactccaagactaatggatgatttcaaggtagggactattgctcacgttattatcagggaaacaaatacctctagcttctcacagatgaataaatgaaaaggcccattttctactgtaacactaaaaaggccttatcttccaaggaaatcatagggagacaaggtcaacttgttgggactgtggtttgcaagccttatcttctgatgtcgctttagcagatagaatgtaattttgatggtaactaaggctcagagtcactttctgtatcattgtccaagttattaggagtatttttcttatgttccgaaatagaagaaagatagtaaagatgagactatgcaaaggattacatggatcaacagtacttattttccaaagatgaggataagatgatgatggtagtggtggcgatggtgtgtgtgtgtgtgcgtgcgtgctaaggtcagtgcaacagaacagaattgttcaaagagaaaaatcacatccacattagattcttcttattgctatcatctctttgaattataaaaataattttgatacagtaaaacctcattaatttggattccactaaccaggagtttgtgagatgaagttacccttacgttaaggaagggcttataaaagcaattttgaaagacacgttttaactacttcaaagagccttttcttttcaagcatttgagaagcacctgtttacttccaattggtgtgctaattataaacttttgatctattcactgaggccaaggttttaagcacttctacagtgaaatgctataatgtcctttttgatattttctctgtgtgccttaaaatattctgtagttgttatttttcactgattcctataagctttcttcaaaattgtatcttattgcatatgaaccacacatgtaattttgggtataataatttatcttgctaagacattgtatacttattgtacagttttatacaacaacatatattacatattcacacaatctacctctttgtatgatgtagaatagtggctgtgaactgggagaaattttggcaatgactggagacattttgattgtcattactaggaggttcttactggcatctagtagacagaggccagggatgttgctaacatcctacaatacacaggacagttccccacaacaaagactttcagctaatagtgctgcttttgagaaatctcgatgtagatcaagttaaaacaagttaaatcttattgaaggcttcagaaatactcatcaaatgtactgctactttggactgaatttcattatttctaaaataaactaatattttactcttttagttttttttaaaatacagaaacgataaagtatttgttctgaaaatcagaaaactaagtctttgaaacagatggtacaaagaatacattgcaatttggccactagtattttctagatcctactcttaagtttctttaatatttttaccatataattttataattctataaattatacagtcatgtaatgtctgtgtttccaagccagattctgttaccgtaaggctgttcacaggagtctgggagattcagagaggctttcttaacaagaggattcaaggactctgagaaatgctatcctagtgtacattatctaactctttcactcatctttgttctcctcaaaattactgagaacattgtaccactagaaacatttgctagaaagtacaacttctagcaaaaaattagactaaaaaggaaataaaaatacgattttttggctaataaaataacctgaaatccaggaaaattgtgaagtcttaagaaacacaaatgtaaatccaatgagaccttgataaacaaaaattcaataagccaaaaccataattaaaacttttcttgacgaaacaacatattacaggatgggtcctggaatgtgtatatatacattcctataacttttgacttccagaatcatgttaaatggtagtaggtgtctctatttggttttgactctggtgcttttctggtgagttatagataccttgtatcatgttaaggatattctttattccagctttaaaagagtctttaataagggacaagtgtttggcatctattgacataatctagtggcttatattatttgacctagggacaaaagcattgattttgtatcattaaactctttatgtatttctattgtctataatgatgactgagaccaagatagcaaacagatcactatattttataaagatttccagtggtaagtatcgaaccaatttccagtggtaagtatcaaaccgaaaggtattttctaaggaaagcccttgtaaatcagaaatgtcataaatcagaatccctttcccaaaacattaactgagattttactgaatcacactaaagagaatgaccagtttggtttgtgaatgtcaggctgcaagagcacctttcgattgcagaccctactgggtttgaacagtaatatactgtgtaactggcagacaaggatacaaatgaagcttttaaaatatatcactttagaagctgaaattggggtgtgtgaaatttccctttttgtgaagtcagttctcatagctaactctattgttcctatagattccccacacctactaccaactcccctatagagtacaagccaggctgaagaaaatgctttgaggtgacccaaccctgcatggtttgtgctaaaaacagcaacccattctgaaggtgatagaaatgaaactgattgtgttgggaataatttactatactggcaatatttgattttgacacaactgtgaatgatgtaaaacatggagagagaacattaatcagactcttgccataagaattcaataaggttctagtacaatgaaagttacagatgaggagaaaactctgggttcttgttttgttttgttttccgtttcagttgggtatggcaaatatatttgaaatgcactgacatcttcaaatgcagattttttaaattgttgagtgtggcccaattgatagaaatagtttaccatgaatctttttttcttctatcacaacatgcttttttttcttttccccttaagatgttaatttatcatgcaaagattttttttcattaagtgcattaatgcttttgtttgtacaggaattttcaaatcaagaggactccccgtagttactaaatataaatccttatcgaatgacatgccaagatgatagctccattccacatgggaaaaggcaaattcagccgtattttgggattttaaccagggctccagcctttgggttgcacagtgtctctgatacatctcttttatgaaaatttcagattgactgtaaatggaacattttgtagaagaaactggcttctagcagttgagtagtgatgctgggaataaatttggtttccctgaatatggtttctcaaagcagtcacagcttctttagaagtcagaattggtaccatttcttatccttgtatttcagcattaactcatgtgcatgtttggaaaatgcttctgcactggtcatcatgcctgcagttttctcttccagctctcctagcctctgtcctctttcatcaagtgcaatccgtgcacgggtcagctctcccatcacccctccagcagcgcctttcatcccttctatactacctggtccaggaatgtgttgcgcaaggctgcgggatgcttttcctgccgaagcttccccaaagagctcttctctgtcaaatgtttgtccgcttccaccaaacagtcccttgagaaagcctctgttttgagcttctggtgtctctatgggagtaaacaaatctcctagcatgtcctgtagattatcacacatttcttggctgtatgttaaccgctgaatttcagtaggagagacgaggtataatgcctgtccttcattggtaaaacaaaatgttcgtgctatcctcatgtctgtcagtggcaaataattaacatccaacattgggcgaagactaggtaggctcattatcatgatatgtccgttagcacaaaagcatgccaagcaggcactgctacacatgaccaccacatttgcttgcagtataaaagatgtctccgtgatgttatgaacataaaggcaagtctgagaaggcagtgagaagactttggcttgtttttctgagcagattattgtatactgatgatctcctatttcttgggatgcagaagatgagttcattaccactttccttctccaagatttttcattttcatctatgttgtttggatccctccaaacttcatatggcggttgcattaatccacccattcggtccatacaggagaatgttagcacagctcctttcaatgagaggaatgtaccacttggcaataccatgactggctctgtaaacctttgttcatctgctaatggtaggtttaaggagatgattaacaccattcccagactggttccaacgaacagacaaggagagatggtagagtcatttttccgtgcaaaggagtccatgaagtatagtgctgtaattgcttctttagaatctttgtcaatactggagatactagagcttctagaacgattataggaattttctcggttttcttctgttgtaactggtaaagaaatctccatgcaggctgctgactgggcctttcgaaatggtggtcttccaggaccccagcgatttacttttgaaacatcggcactagaaagacgttttccagaactgcaactctgagaagttggacttgtgcagtgtccatttacatggtctgaggtaggagacttgcagcgctcaagttctaggggaactggactgtcattcagttcagttaaacctgcaatgaactgtttgttttttcgaggagaccgtggttgtcgctggtataagtcacttgatctatataggtcaatggtccccatgcttaacagtactgtcttctgtataaaatccaccacagccaacccattgcagttcccaaatgcaactattccatatgctgagcttacagcaagactagtaatctgttgtggaggttcaccatctacccacaccaattgaataacaagttctgcttgatatcctggaggcattcgcactggccgtgtcttcacattgaggcatggaatactgtcctttgttactccttcactagcaacagtgttagtgctcccagaaagactccttgaagaaggaagctgggctgagagatctggaaacggaggacttgtttctggttcaggggtaataatatcttcaacatcatactgaagtcgtacctctaatgacactatttctgttgtaatttcatgtctgctgaatttataaattatgacatatgcagagactcctgatacacagaatattctgctctctggacaccagtaaatcatctgaatggcaaatgggtcttcctctacaatttcacatgtttgttttccttctcctaccttctgtttttcaaacacttttgaagtttttagcttgtacagcatctgcagagttattgcagaagcatcccaaaattttattgatccatctgcatgaccagtaataataatttctggatatgtttgtgctccaaggttccaagctcctccactgattggccactccttattactgtatccttgttttttatgcttgactcctatagaatacagtactagaatcaaatccggaggacaatctgcaaagtatgctgtgcatgtaactggtgattcatgaatgtccatgggatatggattttcaaagattggaaaattgctttgtgtcagatcaactacaatgagatctttctccagaagtaccacgacagcatagggttcttgaaattcatttggatagggcgtttcacataaagttagaaattcaacaataggatgatccatttcaagtactgtaattgcttttccatgcatgatggttaaacttggtcttctacaagctttgtcataggacagcccaccagagaatattatgaatggttcgctgtttttgcaggtcttgtattctactttaagaattggtttacaagattcagattttcttccttctctttgactttttccatgtggaattgtggtctggaaagggcgacttgggcttttcaggttccataaagtcaaactaccatctgaatggctgcacatgaactgtttgccctcatgatgccaatcaattgaatgaatagcctcatcataataaactctcagttctgctcttttagatttcaagtcccagaatactacagtaccattttcataacctattagcagtttgccttcatctcttgggctatcgcttaaatgtacaactggacctggatgagtcttagtggatagttcaattgccttgttccacatgataacatatccagaaagaatgaaagattcaatatttacaatatgtgtatttcctctttctgttccaacataaagccatttactctggaaaggtagatgacagtaagtaattcgttcccggttaaatttaagagaatggagtatggctggccttttttgtctaaggttccacaaatgaagtgtatcatctgaacttgcactgaccaaggcaccctcattgatcaaaaattggagctgtaggacagctgcaccactttcatgttggcaatagcaatcaacaccaggtctcccgagtattcgtatagcacctgttctcgtcccaatagccaagattttctgaactggatcaaaggctaatgctgtgggctgatgaggaaaaccatgccgaactgtcttgcaaatctggaaatactccgaagtcaaagtttcctgaatttcctctctgagaacccctgcagtccccgccggatgtacggaaccacttccagccccaccaccactgttactgccactgctgctaccactgccaggggaggaggcagttaagccatccaaaacttttcggaaattaaacttcttcattttaaacactctgcccgcagccgccgccgcgctctcccgcctgttcgcccgcccgccgtccgctctccccgctgcacggcagccgctctcgggggacgtgaagcggtggcggcgacggctgcggcccgagtc

SEQ ID NO: 8890 - RNA, 8420 nt, Homo sapiens
  source 1..8420: mol_type = other RNA
acagcactgcctggtcagaaattctcaaatgcttttgttctgtgagacatacagaataaataccattactatatcttacatcttgccttccctgaccactcagaactggggctggagcaccagccaaggcagacaaacaaggtttccttagttggccataaagcagtgataatcaactttggctggacattagaaccgccttggaggctttcgcaaatattggtgtctggttcccactccaaatgattttaatataattgggaatttaaaaatttcctgaggtgattcttatgtacagtcaaggttgagaatcactcctctagataaatgtgtaaatcaaagcatccatctgtgcatctgattccttaaagcctctttcacttcactgtggctcccatgtccttcctcaccacgatcttcttgcaccaaattggtacttcctcctccttttctaagacagaccttacctattctacatttcatgctttcagggctatgttgtctgcaaatacacacactaaacttgttatgttgacaaccatgttccctggaatggtgcatactagaggtactgctcaaaccaagtacaccacaagtatttctggcacccaggacagtgtgcatgtgaaatagtacctagccaaaaatggagttgcatgacagaggacagaggtgaagaagctgtgaaagccaccacgtttctcctgacacagataccaagacctgatatgaatgttttgacttcttttgcattgccctgtgtgagccaacatggtcaagttacaattcttttttctcatagcagcaggttgtaatcacacagatatactcccagtttgacccaatgatcctaagccaaggagaggatttttagcttacttttctagattggcttcatttttcccttctgcttgaatataagaatctattttaatcttcttcaaccaatgttaggcctaatctgattcttttttctctcaaagtcatggtgatcccttcatgtagataaagtatagatgatgcctttaaaactggtacatgggtcacataaaaagggactccaacagtaaaccttttccttcagatccctagaaactttgagggaaaggagttggattttgatttatttatttgagaatcactttcaaaagatctgagaaaattgtctttgtgactgaatcactggaaaacatctcattcagttctgtcactgtcctttcagagttccagttagacaatgatcttgacaatgattggggccctaaagtctggggctcagtgaagtgtaagaagcaaagtcagtagtactgcttttgtaggtgattaaaacaaatgaggaatcaatcattcctccctccaaactccaagactaatggatgatttcaaggtagggactattgctcacgttattatcagggaaacaaatacctctagcttctcacagatgaataaatgaaaaggcccattttctactgtaacactaaaaaggccttatcttccaaggaaatcatagggagacaaggtcaacttgttgggactgtggtttgcaagccttatcttctgatgtcgctttagcagatagaatgtaattttgatggtaactaaggctcagagtcactttctgtatcattgtccaagttattaggagtatttttcttatgttccgaaatagaagaaagatagtaaagatgagactatgcaaaggattacatggatcaacagtacttattttccaaagatgaggataagatgatgatggtagtggtggcgatggtgtgtgtgtgtgtgcgtgcgtgctaaggtcagtgcaacagaacagaattgttcaaagagaaaaatcacatccacattagattcttcttattgctatcatctctttgaattataaaaataattttgatacagtaaaacctcattaatttggattccactaaccaggagtttgtgagatgaagttacccttacgttaaggaagggcttataaaagcaattttgaaagacacgttttaactacttcaaagagccttttcttttcaagcatttgagaagcacctgtttacttccaattggtgtgctaattataaacttttgatctattcactgaggccaaggttttaagcacttctacagtgaaatgctataatgtcctttttgatattttctctgtgtgccttaaaatattctgtagttgttatttttcactgattcctataagctttcttcaaaattgtatcttattgcatatgaaccacacatgtaattttgggtataataatttatcttgctaagacattgtatacttattgtacagttttatacaacaacatatattacatattcacacaatctacctctttgtatgatgtagaatagtggctgtgaactgggagaaattttggcaatgactggagacattttgattgtcattactaggaggttcttactggcatctagtagacagaggccagggatgttgctaacatcctacaatacacaggacagttccccacaacaaagactttcagctaatagtgctgcttttgagaaatctcgatgtagatcaagttaaaacaagttaaatcttattgaaggcttcagaaatactcatcaaatgtactgctactttggactgaatttcattatttctaaaataaactaatattttactcttttagttttttttaaaatacagaaacgataaagtatttgttctgaaaatcagaaaactaagtctttgaaacagatggtacaaagaatacattgcaatttggccactagtattttctagatcctactcttaagtttctttaatatttttaccatataattttataattctataaattatacagtcatgtaatgtctgtgtttccaagccagattctgttaccgtaaggctgttcacaggagtctgggagattcagagaggctttcttaacaagaggattcaaggactctgagaaatgctatcctagtgtacattatctaactctttcactcatctttgttctcctcaaaattactgagaacattgtaccactagaaacatttgctagaaagtacaacttctagcaaaaaattagactaaaaaggaaataaaaatacgattttttggctaataaaataacctgaaatccaggaaaattgtgaagtcttaagaaacacaaatgtaaatccaatgagaccttgataaacaaaaattcaataagccaaaaccataattaaaacttttcttgacgaaacaacatattacaggatgggtcctggaatgtgtatatatacattcctataacttttgacttccagaatcatgttaaatggtagtaggtgtctctatttggttttgactctggtgcttttctggtgagttatagataccttgtatcatgttaaggatattctttattccagctttaaaagagtctttaataagggacaagtgtttggcatctattgacataatctagtggcttatattatttgacctagggacaaaagcattgattttgtatcattaaactctttatgtatttctattgtctataatgatgactgagaccaagatagcaaacagatcactatattttataaagatttccagtggtaagtatcgaaccaatttccagtggtaagtatcaaaccgaaaggtattttctaaggaaagcccttgtaaatcagaaatgtcataaatcagaatccctttcccaaaacattaactgagattttactgaatcacactaaagagaatgaccagtttggtttgtgaatgtcaggctgcaagagcacctttcgattgcagaccctactgggtttgaacagtaatatactgtgtaactggcagacaaggatacaaatgaagcttttaaaatatatcactttagaagctgaaattggggtgtgtgaaatttccctttttgtgaagtcagttctcatagctaactctattgttcctatagattccccacacctactaccaactcccctatagagtacaagccaggctgaagaaaatgctttgaggtgacccaaccctgcatggtttgtgctaaaaacagcaacccattctgaaggtgatagaaatgaaactgattgtgttgggaataatttactatactggcaatatttgattttgacacaactgtgaatgatgtaaaacatggagagagaacattaatcagactcttgccataagaattcaataaggttctagtacaatgaaagttacagatgaggagaaaactctgggttcttgttttgttttgttttccgtttcagttgggtatggcaaatatatttgaaatgcactgacatcttcaaatgcagattttttaaattgttgagtgtggcccaattgatagaaatagtttaccatgaatctttttttcttctatcacaacatgcttttttttcttttccccttaagatgttaatttatcatgcaaagattttttttcattaagtgcattaatgcttttgtttgtacaggaattttcaaatcaagaggactccccgtagttactaaatataaatccttatcgaatgacatgccaagatgatagctccattccacatgggaaaaggcaaattcagccgtattttgggattttaaccagggctccagcctttgggttgcacagtgtctctgatacatctcttttatgaaaatttcagattgactgtaaatggaacattttgtagaagaaactggcttctagcagttgagtagtgatgctgggaataaatttggtttccctgaatatggtttctcaaagcagtcacagcttctttagaagtcagaattggtaccatttcttatccttgtatttcagcattaactcatgtgcatgtttggaaaatgcttctgcactggtcatcatgcctgcagttttctcttccagctctcctagcctctgtcctctttcatcaagtgcaatccgtgcacgggtcagctctcccatcacccctccagcagcgcctttcatcccttctatactacctggtccaggaatgtgttgcgcaaggctgcgggatgcttttcctgccgaagcttccccaaagagctcttctctgtcaaatgtttgtccgcttccaccaaacagtcccttgagaaagcctctgttttgagcttctggtgtctctatgggagtaaacaaatctcctagcatgtcctgtagattatcacacatttcttggctgtatgttaaccgctgaatttcagtaggagagacgaggtataatgcctgtccttcattggtaaaacaaaatgttcgtgctatcctcatgtctgtcagtggcaaataattaacatccaacattgggcgaagactaggtaggctcattatcatgatatgtccgttagcacaaaagcatgccaagcaggcactgctacacatgaccaccacatttgcttgcagtataaaagatgtctccgtgatgttatgaacataaaggcaagtctgagaaggcagtgagaagactttggcttgtttttctgagcagattattgtatactgatgatctcctatttcttgggatgcagaagatgagttcattaccactttccttctccaagatttttcattttcatctatgttgtttggatccctccaaacttcatatggcggttgcattaatccacccattcggtccatacaggagaatgttagcacagctcctttcaatgagaggaatgtaccacttggcaataccatgactggctctgtaaacctttgttcatctgctaatggtaggtttaaggagatgattaacaccattcccagactggttccaacgaacagacaaggagagatggtagagtcatttttccgtgcaaaggagtccatgaagtatagtgctgtaattgcttctttagaatctttgtcaatactggagatactagagcttctagaacgattataggaattttctcggttttcttctgttgtaactggtaaagaaatctccatgcaggctgctgactgggcctttcgaaatggtggtcttccaggaccccagcgatttacttttgaaacatcggcactagaaagacgttttccagaactgcaactctgagaagttggacttgtgcagtgtccatttacatggtctgaggtaggagacttgcagcgctcaagttctaggggaactggactgtcattcagttcagttaaacctgcaatgaactgtttgttttttcgaggagaccgtggttgtcgctggtataagtcacttgatctatataggtcaatggtccccatgcttaacagtactgtcttctgtataaaatccaccacagccaacccattgcagttcccaaatgcaactattccatatgctgagcttacagcaagactagtaatctgttgtggaggttcaccatctacccacaccaattgaataacaagttctgcttgatatcctggaggcattcgcactggccgtgtcttcacattgaggcatggaatactgtcctttgttactccttcactagcaacagtgttagtgctcccagaaagactccttgaagaaggaagctgggctgagagatctggaaacggaggacttgtttctggttcaggggtaataatatcttcaacatcatactgaagtcgtacctctaatgacactatttctgttgtaatttcatgtctgctgaatttataaattatgacatatgcagagactcctgatacacagaatattctgctctctggacaccagtaaatcatctgaatggcaaatgggtcttcctctacaatttcacatgtttgttttccttctcctaccttctgtttttcaaacacttttgaagtttttagcttgtacagcatctgcagagttattgcagaagcatcccaaaattttattgatccatctgcatgaccagtaataataatttctggatatgtttgtgctccaaggttccaagctcctccactgattggccactccttattactgtatccttgttttttatgcttgactcctatagaatacagtactagaatcaaatccggaggacaatctgcaaagtatgctgtgcatgtaactggtgattcatgaatgtccatgggatatggattttcaaagattggaaaattgctttgtgtcagatcaactacaatgagatctttctccagaagtaccacgacagcatagggttcttgaaattcatttggatagggcgtttcacataaagttagaaattcaacaataggatgatccatttcaagtactgtaattgcttttccatgcatgatggttaaacttggtcttctacaagctttgtcataggacagcccaccagagaatattatgaatggttcgctgtttttgcaggtcttgtattctactttaagaattggtttacaagattcagattttcttccttctctttgactttttccatgtggaattgtggtctggaaagggcgacttgggcttttcaggttccataaagtcaaactaccatctgaatggctgcacatgaactgtttgccctcatgatgccaatcaattgaatgaatagcctcatcataataaactctcagttctgctcttttagatttcaagtcccagaatactacagtaccattttcataacctattagcagtttgccttcatctcttgggctatcgcttaaatgtacaactggacctggatgagtcttagtggatagttcaattgccttgttccacatgataacatatccagaaagaatgaaagattcaatatttacaatatgtgtatttcctctttctgttccaacataaagccatttactctggaaaggtagatgacagtaagtaattcgttcccggttaaatttaagagaatggagtatggctggccttttttgtctaaggttccacaaatgaagtgtatcatctgaacttgcactgaccaaggcaccctcattgatcaaaaattggagctgtaggacagctgcaccactttcatgttggcaatagcaatcaacaccaggtctcccgagtattcgtatagcacctgttctcgtcccaatagccaagattttctgaactggatcaaaggctaatgctgtgggctgatgaggaaaaccatgccgaactgtcttgcaaatctggaaatactccgaagtcaaagtttcctgaatttcctctctgagaacccctgcagtccccgccggatgtacggaaccacttccagccccaccaccactgttactgccactgctgctaccactgccaggggaggaggcagttaagccatccaaaacttttcggaaattaaacttcttcattttaaacacttcctcagacgcctctagccgcctgccagcccgggaagctgagggggccgaggtaggcgggctccggccgcttctctgggccctctggtcgcggcgcctggcgctctccgaggtcctaaccgagcagtc

SEQ ID NO: 8891 - RNA, 6971 nt, Homo sapiens
  source 1..6971: mol_type = other RNA
acagcactgcctggtcagaaattctcaaatgcttttgttctgtgagacatacagaataaataccattactatatcttacatcttgccttccctgaccactcagaactggggctggagcaccagccaaggcagacaaacaaggtttccttagttggccataaagcagtgataatcaactttggctggacattagaaccgccttggaggctttcgcaaatattggtgtctggttcccactccaaatgattttaatataattgggaatttaaaaatttcctgaggtgattcttatgtacagtcaaggttgagaatcactcctctagataaatgtgtaaatcaaagcatccatctgtgcatctgattccttaaagcctctttcacttcactgtggctcccatgtccttcctcaccacgatcttcttgcaccaaattggtacttcctcctccttttctaagacagaccttacctattctacatttcatgctttcagggctatgttgtctgcaaatacacacactaaacttgttatgttgacaaccatgttccctggaatggtgcatactagaggtactgctcaaaccaagtacaccacaagtatttctggcacccaggacagtgtgcatgtgaaatagtacctagccaaaaatggagttgcatgacagaggacagaggtgaagaagctgtgaaagccaccacgtttctcctgacacagataccaagacctgatatgaatgttttgacttcttttgcattgccctgtgtgagccaacatggtcaagttacaattcttttttctcatagcagcaggttgtaatcacacagatatactcccagtttgacccaatgatcctaagccaaggagaggatttttagcttacttttctagattggcttcatttttcccttctgcttgaatataagaatctattttaatcttcttcaaccaatgttaggcctaatctgattcttttttctctcaaagtcatggtgatcccttcatgtagataaagtatagatgatgcctttaaaactggtacatgggtcacataaaaagggactccaacagtaaaccttttccttcagatccctagaaactttgagggaaaggagttggattttgatttatttatttgagaatcactttcaaaagatctgagaaaattgtctttgtgactgaatcactggaaaacatctcattcagttctgtcactgtcctttcagagttccagttagacaatgatcttgacaatgattggggccctaaagtctggggctcagtgaagtgtaagaagcaaagtcagtagtactgcttttgtaggtgattaaaacaaatgaggaatcaatcattcctccctccaaactccaagactaatggatgatttcaaggtagggactattgctcacgttattatcagggaaacaaatacctctagcttctcacagatgaataaatgaaaaggcccattttctactgtaacactaaaaaggccttatcttccaaggaaatcatagggagacaaggtcaacttgttgggactgtggtttgcaagccttatcttctgatgtcgctttagcagatagaatgtaattttgatggtaactaaggctcagagtcactttctgtatcattgtccaagttattaggagtatttttcttatgttccgaaatagaagaaagatagtaaagatgagactatgcaaaggattacatggatcaacagtacttattttccaaagatgaggataagatgatgatggtagtggtggcgatggtgtgtgtgtgtgtgcgtgcgtgctaaggtcagtgcaacagaacagaattgttcaaagagaaaaatcacatccacattagattcttcttattgctatcatctctttgaattataaaaataattttgatacagtaaaacctcattaatttggattccactaaccaggagtttgtgagatgaagttacccttacgttaaggaagggcttataaaagcaattttgaaagacacgttttaactacttcaaagagccttttcttttcaagcatttgagaagcacctgtttacttccaattggtgtgctaattataaacttttgatctattcactgaggccaaggttttaagcacttctacagtgaaatgctataatgtcctttttgatattttctctgtgtgccttaaaatattctgtagttgttatttttcactgattcctataagctttcttcaaaattgtatcttattgcatatgaaccacacatgtaattttgggtataataatttatcttgctaagacattgtatacttattgtacagttttatacaacaacatatattacatattcacacaatctacctctttgtatgatgtagaatagtggctgtgaactgggagaaattttggcaatgactggagacattttgattgtcattactaggaggttcttactggcatctagtagacagaggccagggatgttgctaacatcctacaatacacaggacagttccccacaacaaagactttcagctaatagtgctgcttttgagaaatctcgatgtagatcaagttaaaacaagttaaatcttattgaaggcttcagaaatactcatcaaatgtactgctactttggactgaatttcattatttctaaaataaactaatattttactcttttagttttttttaaaatacagaaacgataaagtatttgttctgaaaatcagaaaactaagtctttgaaacagatggtacaaagaatacattgcaatttggccactagtattttctagatcctactcttaagtttctttaatatttttaccatataattttataattctataaattatacagtcatgtaatgtctgtgtttccaagccagattctgttaccgtaaggctgttcacaggagtctgggagattcagagaggctttcttaacaagaggattcaaggactctgagaaatgctatcctagtgtacattatctaactctttcactcatctttgttctcctcaaaattactgagaacattgtaccactagaaacatttgctagaaagtacaacttctagcaaaaaattagactaaaaaggaaataaaaatacgattttttggctaataaaataacctgaaatccaggaaaattgtgaagtcttaagaaacacaaatgtaaatccaatgagaccttgataaacaaaaattcaataagccaaaaccataattaaaacttttcttgacgaaacaacatattacaggatgggtcctggaatgtgtatatatacattcctataacttttgacttccagaatcatgttaaatggtagtaggtgtctctatttggttttgactctggtgcttttctggtgagttatagataccttgtatcatgttaaggatattctttattccagctttaaaagagtctttaataagggacaagtgtttggcatctattgacataatctagtggcttatattatttgacctagggacaaaagcattgattttgtatcattaaactctttatgtatttctattgtctataatgatgactgagaccaagatagcaaacagatcactatattttataaagatttccagtggtaagtatcgaaccaatttccagtggtaagtatcaaaccgaaaggtattttctaaggaaagcccttgtaaatcagaaatgtcataaatcagaatccctttcccaaaacattaactgagattttactgaatcacactaaagagaatgaccagtttggtttgtgaatgtcaggctgcaagagcacctttcgattgcagaccctactgggtttgaacagtaatatactgtgtaactggcagacaaggatacaaatgaagcttttaaaatatatcactttagaagctgaaattggggtgtgtgaaatttccctttttgtgaagtcagttctcatagctaactctattgttcctatagattccccacacctactaccaactcccctatagagtacaagccaggctgaagaaaatgctttgaggtgacccaaccctgcatggtttgtgctaaaaacagcaacccattctgaaggtgatagaaatgaaactgattgtgttgggaataatttactatactggcaatatttgattttgacacaactgtgaatgatgtaaaacatggagagagaacattaatcagactcttgccataagaattcaataaggttctagtacaatgaaagttacagatgaggagaaaactctgggttcttgttttgttttgttttccgtttcagttgggtatggcaaatatatttgaaatgcactgacatcttcaaatgcagattttttaaattgttgagtgtggcccaattgatagaaatagtttaccatgaatctttttttcttctatcacaacatgcttttttttcttttccccttaagatgttaatttatcatgcaaagattttttttcattaagtgcattaatgcttttgtttgtacaggaattttcaaatcaagaggactccccgtagttactaaatataaatccttatcgaatgacatgccaagatgatagctccattccacatgggaaaaggcaaattcagccgtattttgggattttaaccagggctccagcctttgggttgcacagtgtctctgatacatctcttttatgaaaatttcagattgactgtaaatggaacattttgtagaagaaactggcttctagcagttgagtagtgatgctgggaataaatttggtttccctgaatatggtttctcaaagcagtcacagcttctttagaagtcagaattggtaccatttcttatccttgtatttcagcattaactcatgtgcatgtttggaaaatgcttctgcactggtcatcatgcctgcagttttctcttccagctctcctagcctctgtcctctttcatcaagtgcaatccgtgcacgggtcagctctcccatcacccctccagcagcgcctttcatcccttctatactacctggtccaggaatgtgttgcgcaaggctgcgggatgcttttcctgccgaagcttccccaaagagctcttctctgtcaaatgtttgtccgcttccaccaaacagtcccttgagaaagcctctgttttgagcttctggtgtctctatgggagtaaacaaatctcctagcatgtcctgtagattatcacacatttcttggctgtatgttaaccgctgaatttcagtaggagagacgaggtataatgcctgtccttcattggtaaaacaaaatgttcgtgctatcctcatgtctgtcagtggcaaataattaacatccaacattgggcgaagactaggtaggctcattatcatgatatgtccgttagcacaaaagcatgccaagcaggcactgctacacatgaccaccacatttgcttgcagtataaaagatgtctccgtgatgttatgaacataaaggcaagtctgagaaggcagtgagaagactttggcttgtttttctgagcagattattgtatactgatgatctcctatttcttgggatgcagaagatgagttcattaccactttccttctccaagatttttcattttcatctatgttgtttggatccctccaaacttcatatggcggttgcattaatccacccattcggtccatacaggagaatgttagcacagctcctttcaatgagaggaatgtaccacttggcaataccatgactggctctgtaaacctttgttcatctgctaatggtaggtttaaggagatgattaacaccattcccagactggttccaacgaacagacaaggagagatggtagagtcatttttccgtgcaaaggagtccatgaagtatagtgctgtaattgcttctttagaatctttgtcaatactggagatactagagcttctagaacgattataggaattttctcggttttcttctgttgtaactggtaaagaaatctccatgcaggctgctgactgggcctttcgaaatggtggtcttccaggaccccagcgatttacttttgaaacatcggcactagaaagacgttttccagaactgcaactctgagaagttggacttgtgcagtgtccatttacatggtctgaggtaggagacttgcagcgctcaagttctaggggaactggactgtcattcagttcagttaaactctgataggaagtacggatccgtttcgttaaatcaggataaaagttagacaggccacgcatgcaaaagttgtctgcaatgaactgtttgttttttcgaggagaccgtggttgtcgctggtataagtcacttgatctatataggtcaatggtccccatgcttaacagtactgtcttctgtataaaatccaccacagccaacccattgcagttcccaaatgcaactattccatatgctgagcttacagcaagactagtaatctgttgtggaggttcaccatctacccacaccaattgaataacaagttctgcttgatatcctggaggcattcgcactggccgtgtcttcacattgaggcatggaatactgtcctttgttactccttcactagcaacagtgttagtgctcccagaaagactccttgaagaaggaagctgggctgagagatctggaaacggaggacttgtttctggttcaggggtaataatatcttcaacatcatactgaagtcgtacctctaatgacactatttctgttgtaatttcatgtctgctgaatttataaattatgacatatgcagagactcctgatacacagaatattctgctctctggacaccagtaaatcatctgaatggcaaatgggtcttcctctacaatttcacatgtttgttttccttctcctaccttctgtttttcaaacacttttgaagtttttagcttgtacagcatctgcagagttaccagtaataataatttctggatatgtttgtgctccaaggttccaagctcctccactga

SEQ ID NO: 8892 - RNA, 8569 nt, Homo sapiens
  source 1..8569: mol_type = other RNA
acagcactgcctggtcagaaattctcaaatgcttttgttctgtgagacatacagaataaataccattactatatcttacatcttgccttccctgaccactcagaactggggctggagcaccagccaaggcagacaaacaaggtttccttagttggccataaagcagtgataatcaactttggctggacattagaaccgccttggaggctttcgcaaatattggtgtctggttcccactccaaatgattttaatataattgggaatttaaaaatttcctgaggtgattcttatgtacagtcaaggttgagaatcactcctctagataaatgtgtaaatcaaagcatccatctgtgcatctgattccttaaagcctctttcacttcactgtggctcccatgtccttcctcaccacgatcttcttgcaccaaattggtacttcctcctccttttctaagacagaccttacctattctacatttcatgctttcagggctatgttgtctgcaaatacacacactaaacttgttatgttgacaaccatgttccctggaatggtgcatactagaggtactgctcaaaccaagtacaccacaagtatttctggcacccaggacagtgtgcatgtgaaatagtacctagccaaaaatggagttgcatgacagaggacagaggtgaagaagctgtgaaagccaccacgtttctcctgacacagataccaagacctgatatgaatgttttgacttcttttgcattgccctgtgtgagccaacatggtcaagttacaattcttttttctcatagcagcaggttgtaatcacacagatatactcccagtttgacccaatgatcctaagccaaggagaggatttttagcttacttttctagattggcttcatttttcccttctgcttgaatataagaatctattttaatcttcttcaaccaatgttaggcctaatctgattcttttttctctcaaagtcatggtgatcccttcatgtagataaagtatagatgatgcctttaaaactggtacatgggtcacataaaaagggactccaacagtaaaccttttccttcagatccctagaaactttgagggaaaggagttggattttgatttatttatttgagaatcactttcaaaagatctgagaaaattgtctttgtgactgaatcactggaaaacatctcattcagttctgtcactgtcctttcagagttccagttagacaatgatcttgacaatgattggggccctaaagtctggggctcagtgaagtgtaagaagcaaagtcagtagtactgcttttgtaggtgattaaaacaaatgaggaatcaatcattcctccctccaaactccaagactaatggatgatttcaaggtagggactattgctcacgttattatcagggaaacaaatacctctagcttctcacagatgaataaatgaaaaggcccattttctactgtaacactaaaaaggccttatcttccaaggaaatcatagggagacaaggtcaacttgttgggactgtggtttgcaagccttatcttctgatgtcgctttagcagatagaatgtaattttgatggtaactaaggctcagagtcactttctgtatcattgtccaagttattaggagtatttttcttatgttccgaaatagaagaaagatagtaaagatgagactatgcaaaggattacatggatcaacagtacttattttccaaagatgaggataagatgatgatggtagtggtggcgatggtgtgtgtgtgtgtgcgtgcgtgctaaggtcagtgcaacagaacagaattgttcaaagagaaaaatcacatccacattagattcttcttattgctatcatctctttgaattataaaaataattttgatacagtaaaacctcattaatttggattccactaaccaggagtttgtgagatgaagttacccttacgttaaggaagggcttataaaagcaattttgaaagacacgttttaactacttcaaagagccttttcttttcaagcatttgagaagcacctgtttacttccaattggtgtgctaattataaacttttgatctattcactgaggccaaggttttaagcacttctacagtgaaatgctataatgtcctttttgatattttctctgtgtgccttaaaatattctgtagttgttatttttcactgattcctataagctttcttcaaaattgtatcttattgcatatgaaccacacatgtaattttgggtataataatttatcttgctaagacattgtatacttattgtacagttttatacaacaacatatattacatattcacacaatctacctctttgtatgatgtagaatagtggctgtgaactgggagaaattttggcaatgactggagacattttgattgtcattactaggaggttcttactggcatctagtagacagaggccagggatgttgctaacatcctacaatacacaggacagttccccacaacaaagactttcagctaatagtgctgcttttgagaaatctcgatgtagatcaagttaaaacaagttaaatcttattgaaggcttcagaaatactcatcaaatgtactgctactttggactgaatttcattatttctaaaataaactaatattttactcttttagttttttttaaaatacagaaacgataaagtatttgttctgaaaatcagaaaactaagtctttgaaacagatggtacaaagaatacattgcaatttggccactagtattttctagatcctactcttaagtttctttaatatttttaccatataattttataattctataaattatacagtcatgtaatgtctgtgtttccaagccagattctgttaccgtaaggctgttcacaggagtctgggagattcagagaggctttcttaacaagaggattcaaggactctgagaaatgctatcctagtgtacattatctaactctttcactcatctttgttctcctcaaaattactgagaacattgtaccactagaaacatttgctagaaagtacaacttctagcaaaaaattagactaaaaaggaaataaaaatacgattttttggctaataaaataacctgaaatccaggaaaattgtgaagtcttaagaaacacaaatgtaaatccaatgagaccttgataaacaaaaattcaataagccaaaaccataattaaaacttttcttgacgaaacaacatattacaggatgggtcctggaatgtgtatatatacattcctataacttttgacttccagaatcatgttaaatggtagtaggtgtctctatttggttttgactctggtgcttttctggtgagttatagataccttgtatcatgttaaggatattctttattccagctttaaaagagtctttaataagggacaagtgtttggcatctattgacataatctagtggcttatattatttgacctagggacaaaagcattgattttgtatcattaaactctttatgtatttctattgtctataatgatgactgagaccaagatagcaaacagatcactatattttataaagatttccagtggtaagtatcgaaccaatttccagtggtaagtatcaaaccgaaaggtattttctaaggaaagcccttgtaaatcagaaatgtcataaatcagaatccctttcccaaaacattaactgagattttactgaatcacactaaagagaatgaccagtttggtttgtgaatgtcaggctgcaagagcacctttcgattgcagaccctactgggtttgaacagtaatatactgtgtaactggcagacaaggatacaaatgaagcttttaaaatatatcactttagaagctgaaattggggtgtgtgaaatttccctttttgtgaagtcagttctcatagctaactctattgttcctatagattccccacacctactaccaactcccctatagagtacaagccaggctgaagaaaatgctttgaggtgacccaaccctgcatggtttgtgctaaaaacagcaacccattctgaaggtgatagaaatgaaactgattgtgttgggaataatttactatactggcaatatttgattttgacacaactgtgaatgatgtaaaacatggagagagaacattaatcagactcttgccataagaattcaataaggttctagtacaatgaaagttacagatgaggagaaaactctgggttcttgttttgttttgttttccgtttcagttgggtatggcaaatatatttgaaatgcactgacatcttcaaatgcagattttttaaattgttgagtgtggcccaattgatagaaatagtttaccatgaatctttttttcttctatcacaacatgcttttttttcttttccccttaagatgttaatttatcatgcaaagattttttttcattaagtgcattaatgcttttgtttgtacaggaattttcaaatcaagaggactccccgtagttactaaatataaatccttatcgaatgacatgccaagatgatagctccattccacatgggaaaaggcaaattcagccgtattttgggattttaaccagggctccagcctttgggttgcacagtgtctctgatacatctcttttatgaaaatttcagattgactgtaaatggaacattttgtagaagaaactggcttctagcagttgagtagtgatgctgggaataaatttggtttccctgaatatggtttctcaaagcagtcacagcttctttagaagtcagaattggtaccatttcttatccttgtatttcagcattaactcatgtgcatgtttggaaaatgcttctgcactggtcatcatgcctgcagttttctcttccagctctcctagcctctgtcctctttcatcaagtgcaatccgtgcacgggtcagctctcccatcacccctccagcagcgcctttcatcccttctatactacctggtccaggaatgtgttgcgcaaggctgcgggatgcttttcctgccgaagcttccccaaagagctcttctctgtcaaatgtttgtccgcttccaccaaacagtcccttgagaaagcctctgttttgagcttctggtgtctctatgggagtaaacaaatctcctagcatgtcctgtagattatcacacatttcttggctgtatgttaaccgctgaatttcagtaggagagacgaggtataatgcctgtccttcattggtaaaacaaaatgttcgtgctatcctcatgtctgtcagtggcaaataattaacatccaacattgggcgaagactaggtaggctcattatcatgatatgtccgttagcacaaaagcatgccaagcaggcactgctacacatgaccaccacatttgcttgcagtataaaagatgtctccgtgatgttatgaacataaaggcaagtctgagaaggcagtgagaagactttggcttgtttttctgagcagattattgtatactgatgatctcctatttcttgggatgcagaagatgagttcattaccactttccttctccaagatttttcattttcatctatgttgtttggatccctccaaacttcatatggcggttgcattaatccacccattcggtccatacaggagaatgttagcacagctcctttcaatgagaggaatgtaccacttggcaataccatgactggctctgtaaacctttgttcatctgctaatggtaggtttaaggagatgattaacaccattcccagactggttccaacgaacagacaaggagagatggtagagtcatttttccgtgcaaaggagtccatgaagtatagtgctgtaattgcttctttagaatctttgtcaatactggagatactagagcttctagaacgattataggaattttctcggttttcttctgttgtaactggtaaagaaatctccatgcaggctgctgactgggcctttcgaaatggtggtcttccaggaccccagcgatttacttttgaaacatcggcactagaaagacgttttccagaactgcaactctgagaagttggacttgtgcagtgtccatttacatggtctgaggtaggagacttgcagcgctcaagttctaggggaactggactgtcattcagttcagttaaactctgataggaagtacggatccgtttcgttaaatcaggataaaagttagacaggccacgcatgcaaaagttgtctgcaatgaactgtttgttttttcgaggagaccgtggttgtcgctggtataagtcacttgatctatataggtcaatggtccccatgcttaacagtactgtcttctgtataaaatccaccacagccaacccattgcagttcccaaatgcaactattccatatgctgagcttacagcaagactagtaatctgttgtggaggttcaccatctacccacaccaattgaataacaagttctgcttgatatcctggaggcattcgcactggccgtgtcttcacattgaggcatggaatactgtcctttgttactccttcactagcaacagtgttagtgctcccagaaagactccttgaagaaggaagctgggctgagagatctggaaacggaggacttgtttctggttcaggggtaataatatcttcaacatcatactgaagtcgtacctctaatgacactatttctgttgtaatttcatgtctgctgaatttataaattatgacatatgcagagactcctgatacacagaatattctgctctctggacaccagtaaatcatctgaatggcaaatgggtcttcctctacaatttcacatgtttgttttccttctcctaccttctgtttttcaaacacttttgaagtttttagcttgtacagcatctgcagagttattgcagaagcatcccaaaattttattgatccatctgcatgaccagtaataataatttctggatatgtttgtgctccaaggttccaagctcctccactgattggccactccttattactgtatccttgttttttatgcttgactcctatagaatacagtactagaatcaaatccggaggacaatctgcaaagtatgctgtgcatgtaactggtgattcatgaatgtccatgggatatggattttcaaagattggaaaattgctttgtgtcagatcaactacaatgagatctttctccagaagtaccacgacagcatagggttcttgaaattcatttggatagggcgtttcacataaagttagaaattcaacaataggatgatccatttcaagtactgtaattgcttttccatgcatgatggttaaacttggtcttctacaagctttgtcataggacagcccaccagagaatattatgaatggttcgctgtttttgcaggtcttgtattctactttaagaattggtttacaagattcagattttcttccttctctttgactttttccatgtggaattgtggtctggaaagggcgacttgggcttttcaggttccataaagtcaaactaccatctgaatggctgcacatgaactgtttgccctcatgatgccaatcaattgaatgaatagcctcatcataataaactctcagttctgctcttttagatttcaagtcccagaatactacagtaccattttcataacctattagcaggtgattatgaaggctgacaagtcccaagatctgcagggtgagctggcaagcaggagatccaggagagctgatggtgtgccagtctgagtctgaagactttgccttcatctcttgggctatcgcttaaatgtacaactggacctggatgagtcttagtggatagttcaattgccttgttccacatgataacatatccagaaagaatgaaagattcaatatttacaatatgtgtatttcctctttctgttccaacataaagccatttactctggaaaggtagatgacagtaagtaattcgttcccggttaaatttaagagaatggagtatggctggccttttttgtctaaggttccacaaatgaagtgtatcatctgaacttgcactgaccaaggcaccctcattgatcaaaaattggagctgtaggacagctgcaccactttcatgttggcaatagcaatcaacaccaggtctcccgagtattcgtatagcacctgttctcgtcccaatagccaagattttctgaactggatcaaaggctaatgctgtgggctgatgaggaaaaccatgccgaactgtcttgcaaatctggaaatactccgaagtcaaagtttcctgaatttcctctctgagaacccctgcagtccccgccggatgtacggaaccacttccagccccaccaccactgttactgccactgctgctaccactgccaggggaggaggcagttaagccatccaaaacttttcggaaattaaacttcttcattttaaacacttcctcagacgcctctagccgcctgccagcccgggaagctgagggggccgaggtaggcgggctccggccgcttctctgggccctctggtcgcggcgcctggcgctctcc

SEQ ID NO: 8893 - RNA, 8664 nt, Homo sapiens
  source 1..8664: mol_type = other RNA
acagcactgcctggtcagaaattctcaaatgcttttgttctgtgagacatacagaataaataccattactatatcttacatcttgccttccctgaccactcagaactggggctggagcaccagccaaggcagacaaacaaggtttccttagttggccataaagcagtgataatcaactttggctggacattagaaccgccttggaggctttcgcaaatattggtgtctggttcccactccaaatgattttaatataattgggaatttaaaaatttcctgaggtgattcttatgtacagtcaaggttgagaatcactcctctagataaatgtgtaaatcaaagcatccatctgtgcatctgattccttaaagcctctttcacttcactgtggctcccatgtccttcctcaccacgatcttcttgcaccaaattggtacttcctcctccttttctaagacagaccttacctattctacatttcatgctttcagggctatgttgtctgcaaatacacacactaaacttgttatgttgacaaccatgttccctggaatggtgcatactagaggtactgctcaaaccaagtacaccacaagtatttctggcacccaggacagtgtgcatgtgaaatagtacctagccaaaaatggagttgcatgacagaggacagaggtgaagaagctgtgaaagccaccacgtttctcctgacacagataccaagacctgatatgaatgttttgacttcttttgcattgccctgtgtgagccaacatggtcaagttacaattcttttttctcatagcagcaggttgtaatcacacagatatactcccagtttgacccaatgatcctaagccaaggagaggatttttagcttacttttctagattggcttcatttttcccttctgcttgaatataagaatctattttaatcttcttcaaccaatgttaggcctaatctgattcttttttctctcaaagtcatggtgatcccttcatgtagataaagtatagatgatgcctttaaaactggtacatgggtcacataaaaagggactccaacagtaaaccttttccttcagatccctagaaactttgagggaaaggagttggattttgatttatttatttgagaatcactttcaaaagatctgagaaaattgtctttgtgactgaatcactggaaaacatctcattcagttctgtcactgtcctttcagagttccagttagacaatgatcttgacaatgattggggccctaaagtctggggctcagtgaagtgtaagaagcaaagtcagtagtactgcttttgtaggtgattaaaacaaatgaggaatcaatcattcctccctccaaactccaagactaatggatgatttcaaggtagggactattgctcacgttattatcagggaaacaaatacctctagcttctcacagatgaataaatgaaaaggcccattttctactgtaacactaaaaaggccttatcttccaaggaaatcatagggagacaaggtcaacttgttgggactgtggtttgcaagccttatcttctgatgtcgctttagcagatagaatgtaattttgatggtaactaaggctcagagtcactttctgtatcattgtccaagttattaggagtatttttcttatgttccgaaatagaagaaagatagtaaagatgagactatgcaaaggattacatggatcaacagtacttattttccaaagatgaggataagatgatgatggtagtggtggcgatggtgtgtgtgtgtgtgcgtgcgtgctaaggtcagtgcaacagaacagaattgttcaaagagaaaaatcacatccacattagattcttcttattgctatcatctctttgaattataaaaataattttgatacagtaaaacctcattaatttggattccactaaccaggagtttgtgagatgaagttacccttacgttaaggaagggcttataaaagcaattttgaaagacacgttttaactacttcaaagagccttttcttttcaagcatttgagaagcacctgtttacttccaattggtgtgctaattataaacttttgatctattcactgaggccaaggttttaagcacttctacagtgaaatgctataatgtcctttttgatattttctctgtgtgccttaaaatattctgtagttgttatttttcactgattcctataagctttcttcaaaattgtatcttattgcatatgaaccacacatgtaattttgggtataataatttatcttgctaagacattgtatacttattgtacagttttatacaacaacatatattacatattcacacaatctacctctttgtatgatgtagaatagtggctgtgaactgggagaaattttggcaatgactggagacattttgattgtcattactaggaggttcttactggcatctagtagacagaggccagggatgttgctaacatcctacaatacacaggacagttccccacaacaaagactttcagctaatagtgctgcttttgagaaatctcgatgtagatcaagttaaaacaagttaaatcttattgaaggcttcagaaatactcatcaaatgtactgctactttggactgaatttcattatttctaaaataaactaatattttactcttttagttttttttaaaatacagaaacgataaagtatttgttctgaaaatcagaaaactaagtctttgaaacagatggtacaaagaatacattgcaatttggccactagtattttctagatcctactcttaagtttctttaatatttttaccatataattttataattctataaattatacagtcatgtaatgtctgtgtttccaagccagattctgttaccgtaaggctgttcacaggagtctgggagattcagagaggctttcttaacaagaggattcaaggactctgagaaatgctatcctagtgtacattatctaactctttcactcatctttgttctcctcaaaattactgagaacattgtaccactagaaacatttgctagaaagtacaacttctagcaaaaaattagactaaaaaggaaataaaaatacgattttttggctaataaaataacctgaaatccaggaaaattgtgaagtcttaagaaacacaaatgtaaatccaatgagaccttgataaacaaaaattcaataagccaaaaccataattaaaacttttcttgacgaaacaacatattacaggatgggtcctggaatgtgtatatatacattcctataacttttgacttccagaatcatgttaaatggtagtaggtgtctctatttggttttgactctggtgcttttctggtgagttatagataccttgtatcatgttaaggatattctttattccagctttaaaagagtctttaataagggacaagtgtttggcatctattgacataatctagtggcttatattatttgacctagggacaaaagcattgattttgtatcattaaactctttatgtatttctattgtctataatgatgactgagaccaagatagcaaacagatcactatattttataaagatttccagtggtaagtatcgaaccaatttccagtggtaagtatcaaaccgaaaggtattttctaaggaaagcccttgtaaatcagaaatgtcataaatcagaatccctttcccaaaacattaactgagattttactgaatcacactaaagagaatgaccagtttggtttgtgaatgtcaggctgcaagagcacctttcgattgcagaccctactgggtttgaacagtaatatactgtgtaactggcagacaaggatacaaatgaagcttttaaaatatatcactttagaagctgaaattggggtgtgtgaaatttccctttttgtgaagtcagttctcatagctaactctattgttcctatagattccccacacctactaccaactcccctatagagtacaagccaggctgaagaaaatgctttgaggtgacccaaccctgcatggtttgtgctaaaaacagcaacccattctgaaggtgatagaaatgaaactgattgtgttgggaataatttactatactggcaatatttgattttgacacaactgtgaatgatgtaaaacatggagagagaacattaatcagactcttgccataagaattcaataaggttctagtacaatgaaagttacagatgaggagaaaactctgggttcttgttttgttttgttttccgtttcagttgggtatggcaaatatatttgaaatgcactgacatcttcaaatgcagattttttaaattgttgagtgtggcccaattgatagaaatagtttaccatgaatctttttttcttctatcacaacatgcttttttttcttttccccttaagatgttaatttatcatgcaaagattttttttcattaagtgcattaatgcttttgtttgtacaggaattttcaaatcaagaggactccccgtagttactaaatataaatccttatcgaatgacatgccaagatgatagctccattccacatgggaaaaggcaaattcagccgtattttgggattttaaccagggctccagcctttgggttgcacagtgtctctgatacatctcttttatgaaaatttcagattgactgtaaatggaacattttgtagaagaaactggcttctagcagttgagtagtgatgctgggaataaatttggtttccctgaatatggtttctcaaagcagtcacagcttctttagaagtcagaattggtaccatttcttatccttgtatttcagcattaactcatgtgcatgtttggaaaatgcttctgcactggtcatcatgcctgcagttttctcttccagctctcctagcctctgtcctctttcatcaagtgcaatccgtgcacgggtcagctctcccatcacccctccagcagcgcctttcatcccttctatactacctggtccaggaatgtgttgcgcaaggctgcgggatgcttttcctgccgaagcttccccaaagagctcttctctgtcaaatgtttgtccgcttccaccaaacagtcccttgagaaagcctctgttttgagcttctggtgtctctatgggagtaaacaaatctcctagcatgtcctgtagattatcacacatttcttggctgtatgttaaccgctgaatttcagtaggagagacgaggtataatgcctgtccttcattggtaaaacaaaatgttcgtgctatcctcatgtctgtcagtggcaaataattaacatccaacattgggcgaagactaggtaggctcattatcatgatatgtccgttagcacaaaagcatgccaagcaggcactgctacacatgaccaccacatttgcttgcagtataaaagatgtctccgtgatgttatgaacataaaggcaagtctgagaaggcagtgagaagactttggcttgtttttctgagcagattattgtatactgatgatctcctatttcttgggatgcagaagatgagttcattaccactttccttctccaagatttttcattttcatctatgttgtttggatccctccaaacttcatatggcggttgcattaatccacccattcggtccatacaggagaatgttagcacagctcctttcaatgagaggaatgtaccacttggcaataccatgactggctctgtaaacctttgttcatctgctaatggtaggtttaaggagatgattaacaccattcccagactggttccaacgaacagacaaggagagatggtagagtcatttttccgtgcaaaggagtccatgaagtatagtgctgtaattgcttctttagaatctttgtcaatactggagatactagagcttctagaacgattataggaattttctcggttttcttctgttgtaactggtaaagaaatctccatgcaggctgctgactgggcctttcgaaatggtggtcttccaggaccccagcgatttacttttgaaacatcggcactagaaagacgttttccagaactgcaactctgagaagttggacttgtgcagtgtccatttacatggtctgaggtaggagacttgcagcgctcaagttctaggggaactggactgtcattcagttcagttaaactctgataggaagtacggatccgtttcgttaaatcaggataaaagttagacaggccacgcatgcaaaagttgtctgcaatgaactgtttgttttttcgaggagaccgtggttgtcgctggtataagtcacttgatctatataggtcaatggtccccatgcttaacagtactgtcttctgtataaaatccaccacagccaacccattgcagttcccaaatgcaactattccatatgctgagcttacagcaagactagtaatctgttgtggaggttcaccatctacccacaccaattgaataacaagttctgcttgatatcctggaggcattcgcactggccgtgtcttcacattgaggcatggaatactgtcctttgttactccttcactagcaacagtgttagtgctcccagaaagactccttgaagaaggaagctgggctgagagatctggaaacggaggacttgtttctggttcaggggtaataatatcttcaacatcatactgaagtcgtacctctaatgacactatttctgttgtaatttcatgtctgctgaatttataaattatgacatatgcagagactcctgatacacagaatattctgctctctggacaccagtaaatcatctgaatggcaaatgggtcttcctctacaatttcacatgtttgttttccttctcctaccttctgtttttcaaacacttttgaagtttttagcttgtacagcatctgcagagttattgcagaagcatcccaaaattttattgatccatctgcatgaccagtaataataatttctggatatgtttgtgctccaaggttccaagctcctccactgattggccactccttattactgtatccttgttttttatgcttgactcctatagaatacagtactagaatcaaatccggaggacaatctgcaaagtatgctgtgcatgtaactggtgattcatgaatgtccatgggatatggattttcaaagattggaaaattgctttgtgtcagatcaactacaatgagatctttctccagaagtaccacgacagcatagggttcttgaaattcatttggatagggcgtttcacataaagttagaaattcaacaataggatgatccatttcaagtactgtaattgcttttccatgcatgatggttaaacttggtcttctacaagctttgtcataggacagcccaccagagaatattatgaatggttcgctgtttttgcaggtcttgtattctactttaagaattggtttacaagattcagattttcttccttctctttgactttttccatgtggaattgtggtctggaaagggcgacttgggcttttcaggttccataaagtcaaactaccatctgaatggctgcacatgaactgtttgccctcatgatgccaatcaattgaatgaatagcctcatcataataaactctcagttctgctcttttagatttcaagtcccagaatactacagtaccattttcataacctattagcagtttgccttcatctcttgggctatcgcttaaatgtacaactggacctggatgagtcttagtggatagttcaattgccttgttccacatgataacatatccagaaagaatgaaagattcaatatttacaatatgtgtatttcctctttctgttccaacataaagccatttactctggaaaggtagatgacagtaagtaattcgttcccggttaaatttaagagaatggagtatggctggccttttttgtctaaggttccacaaatgaagtgtatcatctgaacttgcactgaccaaggcaccctcattgatcaaaaattggagctgtaggacagctgcaccactttcatgttggcaatagcaatcaacaccaggtctcccgagtattcgtatagcacctgttctcgtcccaatagccaagattttctgaactggatcaaaggctaatgctgtgggctgatgaggaaaaccatgccgaactgtcttgcaaatctggaaatactccgaagtcaaagtttcctgaatttcctctctgagaacccctgcagtccccgccggatgtacggaaccacttccagccccaccaccactgttactgccactgctgctaccactgccaggggaggaggcagttaagccatccaaaacttttcggaaattaaacttcttcattttaaacacaagactctgtctctctcttaagggcggactttccttcttcgaaacgttcggctcagagtattttattttcagaaaaacgacgttgggggagccggtatttactctgccaccaccttccgggctcttcccccatcagcttcaacgcttccttttttgtcactatgaaaggcggggaggggggtactttttctagtccccatcccccagcagcccggaccccaaaacatctgcgagtgacccacagcaacagctgccggggagggggggaggaggagaacggcgacaccgtctgtttccactt

SEQ ID NO: 8894 - RNA, 8486 nt, Homo sapiens
  source 1..8486: mol_type = other RNA
acagcactgcctggtcagaaattctcaaatgcttttgttctgtgagacatacagaataaataccattactatatcttacatcttgccttccctgaccactcagaactggggctggagcaccagccaaggcagacaaacaaggtttccttagttggccataaagcagtgataatcaactttggctggacattagaaccgccttggaggctttcgcaaatattggtgtctggttcccactccaaatgattttaatataattgggaatttaaaaatttcctgaggtgattcttatgtacagtcaaggttgagaatcactcctctagataaatgtgtaaatcaaagcatccatctgtgcatctgattccttaaagcctctttcacttcactgtggctcccatgtccttcctcaccacgatcttcttgcaccaaattggtacttcctcctccttttctaagacagaccttacctattctacatttcatgctttcagggctatgttgtctgcaaatacacacactaaacttgttatgttgacaaccatgttccctggaatggtgcatactagaggtactgctcaaaccaagtacaccacaagtatttctggcacccaggacagtgtgcatgtgaaatagtacctagccaaaaatggagttgcatgacagaggacagaggtgaagaagctgtgaaagccaccacgtttctcctgacacagataccaagacctgatatgaatgttttgacttcttttgcattgccctgtgtgagccaacatggtcaagttacaattcttttttctcatagcagcaggttgtaatcacacagatatactcccagtttgacccaatgatcctaagccaaggagaggatttttagcttacttttctagattggcttcatttttcccttctgcttgaatataagaatctattttaatcttcttcaaccaatgttaggcctaatctgattcttttttctctcaaagtcatggtgatcccttcatgtagataaagtatagatgatgcctttaaaactggtacatgggtcacataaaaagggactccaacagtaaaccttttccttcagatccctagaaactttgagggaaaggagttggattttgatttatttatttgagaatcactttcaaaagatctgagaaaattgtctttgtgactgaatcactggaaaacatctcattcagttctgtcactgtcctttcagagttccagttagacaatgatcttgacaatgattggggccctaaagtctggggctcagtgaagtgtaagaagcaaagtcagtagtactgcttttgtaggtgattaaaacaaatgaggaatcaatcattcctccctccaaactccaagactaatggatgatttcaaggtagggactattgctcacgttattatcagggaaacaaatacctctagcttctcacagatgaataaatgaaaaggcccattttctactgtaacactaaaaaggccttatcttccaaggaaatcatagggagacaaggtcaacttgttgggactgtggtttgcaagccttatcttctgatgtcgctttagcagatagaatgtaattttgatggtaactaaggctcagagtcactttctgtatcattgtccaagttattaggagtatttttcttatgttccgaaatagaagaaagatagtaaagatgagactatgcaaaggattacatggatcaacagtacttattttccaaagatgaggataagatgatgatggtagtggtggcgatggtgtgtgtgtgtgtgcgtgcgtgctaaggtcagtgcaacagaacagaattgttcaaagagaaaaatcacatccacattagattcttcttattgctatcatctctttgaattataaaaataattttgatacagtaaaacctcattaatttggattccactaaccaggagtttgtgagatgaagttacccttacgttaaggaagggcttataaaagcaattttgaaagacacgttttaactacttcaaagagccttttcttttcaagcatttgagaagcacctgtttacttccaattggtgtgctaattataaacttttgatctattcactgaggccaaggttttaagcacttctacagtgaaatgctataatgtcctttttgatattttctctgtgtgccttaaaatattctgtagttgttatttttcactgattcctataagctttcttcaaaattgtatcttattgcatatgaaccacacatgtaattttgggtataataatttatcttgctaagacattgtatacttattgtacagttttatacaacaacatatattacatattcacacaatctacctctttgtatgatgtagaatagtggctgtgaactgggagaaattttggcaatgactggagacattttgattgtcattactaggaggttcttactggcatctagtagacagaggccagggatgttgctaacatcctacaatacacaggacagttccccacaacaaagactttcagctaatagtgctgcttttgagaaatctcgatgtagatcaagttaaaacaagttaaatcttattgaaggcttcagaaatactcatcaaatgtactgctactttggactgaatttcattatttctaaaataaactaatattttactcttttagttttttttaaaatacagaaacgataaagtatttgttctgaaaatcagaaaactaagtctttgaaacagatggtacaaagaatacattgcaatttggccactagtattttctagatcctactcttaagtttctttaatatttttaccatataattttataattctataaattatacagtcatgtaatgtctgtgtttccaagccagattctgttaccgtaaggctgttcacaggagtctgggagattcagagaggctttcttaacaagaggattcaaggactctgagaaatgctatcctagtgtacattatctaactctttcactcatctttgttctcctcaaaattactgagaacattgtaccactagaaacatttgctagaaagtacaacttctagcaaaaaattagactaaaaaggaaataaaaatacgattttttggctaataaaataacctgaaatccaggaaaattgtgaagtcttaagaaacacaaatgtaaatccaatgagaccttgataaacaaaaattcaataagccaaaaccataattaaaacttttcttgacgaaacaacatattacaggatgggtcctggaatgtgtatatatacattcctataacttttgacttccagaatcatgttaaatggtagtaggtgtctctatttggttttgactctggtgcttttctggtgagttatagataccttgtatcatgttaaggatattctttattccagctttaaaagagtctttaataagggacaagtgtttggcatctattgacataatctagtggcttatattatttgacctagggacaaaagcattgattttgtatcattaaactctttatgtatttctattgtctataatgatgactgagaccaagatagcaaacagatcactatattttataaagatttccagtggtaagtatcgaaccaatttccagtggtaagtatcaaaccgaaaggtattttctaaggaaagcccttgtaaatcagaaatgtcataaatcagaatccctttcccaaaacattaactgagattttactgaatcacactaaagagaatgaccagtttggtttgtgaatgtcaggctgcaagagcacctttcgattgcagaccctactgggtttgaacagtaatatactgtgtaactggcagacaaggatacaaatgaagcttttaaaatatatcactttagaagctgaaattggggtgtgtgaaatttccctttttgtgaagtcagttctcatagctaactctattgttcctatagattccccacacctactaccaactcccctatagagtacaagccaggctgaagaaaatgctttgaggtgacccaaccctgcatggtttgtgctaaaaacagcaacccattctgaaggtgatagaaatgaaactgattgtgttgggaataatttactatactggcaatatttgattttgacacaactgtgaatgatgtaaaacatggagagagaacattaatcagactcttgccataagaattcaataaggttctagtacaatgaaagttacagatgaggagaaaactctgggttcttgttttgttttgttttccgtttcagttgggtatggcaaatatatttgaaatgcactgacatcttcaaatgcagattttttaaattgttgagtgtggcccaattgatagaaatagtttaccatgaatctttttttcttctatcacaacatgcttttttttcttttccccttaagatgttaatttatcatgcaaagattttttttcattaagtgcattaatgcttttgtttgtacaggaattttcaaatcaagaggactccccgtagttactaaatataaatccttatcgaatgacatgccaagatgatagctccattccacatgggaaaaggcaaattcagccgtattttgggattttaaccagggctccagcctttgggttgcacagtgtctctgatacatctcttttatgaaaatttcagattgactgtaaatggaacattttgtagaagaaactggcttctagcagttgagtagtgatgctgggaataaatttggtttccctgaatatggtttctcaaagcagtcacagcttctttagaagtcagaattggtaccatttcttatccttgtatttcagcattaactcatgtgcatgtttggaaaatgcttctgcactggtcatcatgcctgcagttttctcttccagctctcctagcctctgtcctctttcatcaagtgcaatccgtgcacgggtcagctctcccatcacccctccagcagcgcctttcatcccttctatactacctggtccaggaatgtgttgcgcaaggctgcgggatgcttttcctgccgaagcttccccaaagagctcttctctgtcaaatgtttgtccgcttccaccaaacagtcccttgagaaagcctctgttttgagcttctggtgtctctatgggagtaaacaaatctcctagcatgtcctgtagattatcacacatttcttggctgtatgttaaccgctgaatttcagtaggagagacgaggtataatgcctgtccttcattggtaaaacaaaatgttcgtgctatcctcatgtctgtcagtggcaaataattaacatccaacattgggcgaagactaggtaggctcattatcatgatatgtccgttagcacaaaagcatgccaagcaggcactgctacacatgaccaccacatttgcttgcagtataaaagatgtctccgtgatgttatgaacataaaggcaagtctgagaaggcagtgagaagactttggcttgtttttctgagcagattattgtatactgatgatctcctatttcttgggatgcagaagatgagttcattaccactttccttctccaagatttttcattttcatctatgttgtttggatccctccaaacttcatatggcggttgcattaatccacccattcggtccatacaggagaatgttagcacagctcctttcaatgagaggaatgtaccacttggcaataccatgactggctctgtaaacctttgttcatctgctaatggtaggtttaaggagatgattaacaccattcccagactggttccaacgaacagacaaggagagatggtagagtcatttttccgtgcaaaggagtccatgaagtatagtgctgtaattgcttctttagaatctttgtcaatactggagatactagagcttctagaacgattataggaattttctcggttttcttctgttgtaactggtaaagaaatctccatgcaggctgctgactgggcctttcgaaatggtggtcttccaggaccccagcgatttacttttgaaacatcggcactagaaagacgttttccagaactgcaactctgagaagttggacttgtgcagtgtccatttacatggtctgaggtaggagacttgcagcgctcaagttctaggggaactggactgtcattcagttcagttaaactctgataggaagtacggatccgtttcgttaaatcaggataaaagttagacaggccacgcatgcaaaagttgtctgcaatgaactgtttgttttttcgaggagaccgtggttgtcgctggtataagtcacttgatctatataggtcaatggtccccatgcttaacagtactgtcttctgtataaaatccaccacagccaacccattgcagttcccaaatgcaactattccatatgctgagcttacagcaagactagtaatctgttgtggaggttcaccatctacccacaccaattgaataacaagttctgcttgatatcctggaggcattcgcactggccgtgtcttcacattgaggcatggaatactgtcctttgttactccttcactagcaacagtgttagtgctcccagaaagactccttgaagaaggaagctgggctgagagatctggaaacggaggacttgtttctggttcaggggtaataatatcttcaacatcatactgaagtcgtacctctaatgacactatttctgttgtaatttcatgtctgctgaatttataaattatgacatatgcagagactcctgatacacagaatattctgctctctggacaccagtaaatcatctgaatggcaaatgggtcttcctctacaatttcacatgtttgttttccttctcctaccttctgtttttcaaacacttttgaagtttttagcttgtacagcatctgcagagttattgcagaagcatcccaaaattttattgatccatctgcatgaccagtaataataatttctggatatgtttgtgctccaaggttccaagctcctccactgattggccactccttattactgtatccttgttttttatgcttgactcctatagaatacagtactagaatcaaatccggaggacaatctgcaaagtatgctgtgcatgtaactggtgattcatgaatgtccatgggatatggattttcaaagattggaaaattgctttgtgtcagatcaactacaatgagatctttctccagaagtaccacgacagcatagggttcttgaaattcatttggatagggcgtttcacataaagttagaaattcaacaataggatgatccatttcaagtactgtaattgcttttccatgcatgatggttaaacttggtcttctacaagctttgtcataggacagcccaccagagaatattatgaatggttcgctgtttttgcaggtcttgtattctactttaagaattggtttacaagattcagattttcttccttctctttgactttttccatgtggaattgtggtctggaaagggcgacttgggcttttcaggttccataaagtcaaactaccatctgaatggctgcacatgaactgtttgccctcatgatgccaatcaattgaatgaatagcctcatcataataaactctcagttctgctcttttagatttcaagtcccagaatactacagtaccattttcataacctattagcagtttgccttcatctcttgggctatcgcttaaatgtacaactggacctggatgagtcttagtggatagttcaattgccttgttccacatgataacatatccagaaagaatgaaagattcaatatttacaatatgtgtatttcctctttctgttccaacataaagccatttactctggaaaggtagatgacagtaagtaattcgttcccggttaaatttaagagaatggagtatggctggccttttttgtctaaggttccacaaatgaagtgtatcatctgaacttgcactgaccaaggcaccctcattgatcaaaaattggagctgtaggacagctgcaccactttcatgttggcaatagcaatcaacaccaggtctcccgagtattcgtatagcacctgttctcgtcccaatagccaagattttctgaactggatcaaaggctaatgctgtgggctgatgaggaaaaccatgccgaactgtcttgcaaatctggaaatactccgaagtcaaagtttcctgaatttcctctctgagaacccctgcagtccccgccggatgtacggaaccacttccagccccaccaccactgttactgccactgctgctaccactgccaggggaggaggcagttaagccatccaaaacttttcggaaattaaacttcttcattttaaacactctgcccgcagccgccgccgcgctctcccgcctgttcgcccgcccgccgtccgctctccccgctgcacggcagccgctctcgggggacgtgaagcggtggcggcgacggctgcggcccgagtc

SEQ ID NO: 8895 - RNA, 8492 nt, Homo sapiens
  source 1..8492: mol_type = other RNA
acagcactgcctggtcagaaattctcaaatgcttttgttctgtgagacatacagaataaataccattactatatcttacatcttgccttccctgaccactcagaactggggctggagcaccagccaaggcagacaaacaaggtttccttagttggccataaagcagtgataatcaactttggctggacattagaaccgccttggaggctttcgcaaatattggtgtctggttcccactccaaatgattttaatataattgggaatttaaaaatttcctgaggtgattcttatgtacagtcaaggttgagaatcactcctctagataaatgtgtaaatcaaagcatccatctgtgcatctgattccttaaagcctctttcacttcactgtggctcccatgtccttcctcaccacgatcttcttgcaccaaattggtacttcctcctccttttctaagacagaccttacctattctacatttcatgctttcagggctatgttgtctgcaaatacacacactaaacttgttatgttgacaaccatgttccctggaatggtgcatactagaggtactgctcaaaccaagtacaccacaagtatttctggcacccaggacagtgtgcatgtgaaatagtacctagccaaaaatggagttgcatgacagaggacagaggtgaagaagctgtgaaagccaccacgtttctcctgacacagataccaagacctgatatgaatgttttgacttcttttgcattgccctgtgtgagccaacatggtcaagttacaattcttttttctcatagcagcaggttgtaatcacacagatatactcccagtttgacccaatgatcctaagccaaggagaggatttttagcttacttttctagattggcttcatttttcccttctgcttgaatataagaatctattttaatcttcttcaaccaatgttaggcctaatctgattcttttttctctcaaagtcatggtgatcccttcatgtagataaagtatagatgatgcctttaaaactggtacatgggtcacataaaaagggactccaacagtaaaccttttccttcagatccctagaaactttgagggaaaggagttggattttgatttatttatttgagaatcactttcaaaagatctgagaaaattgtctttgtgactgaatcactggaaaacatctcattcagttctgtcactgtcctttcagagttccagttagacaatgatcttgacaatgattggggccctaaagtctggggctcagtgaagtgtaagaagcaaagtcagtagtactgcttttgtaggtgattaaaacaaatgaggaatcaatcattcctccctccaaactccaagactaatggatgatttcaaggtagggactattgctcacgttattatcagggaaacaaatacctctagcttctcacagatgaataaatgaaaaggcccattttctactgtaacactaaaaaggccttatcttccaaggaaatcatagggagacaaggtcaacttgttgggactgtggtttgcaagccttatcttctgatgtcgctttagcagatagaatgtaattttgatggtaactaaggctcagagtcactttctgtatcattgtccaagttattaggagtatttttcttatgttccgaaatagaagaaagatagtaaagatgagactatgcaaaggattacatggatcaacagtacttattttccaaagatgaggataagatgatgatggtagtggtggcgatggtgtgtgtgtgtgtgcgtgcgtgctaaggtcagtgcaacagaacagaattgttcaaagagaaaaatcacatccacattagattcttcttattgctatcatctctttgaattataaaaataattttgatacagtaaaacctcattaatttggattccactaaccaggagtttgtgagatgaagttacccttacgttaaggaagggcttataaaagcaattttgaaagacacgttttaactacttcaaagagccttttcttttcaagcatttgagaagcacctgtttacttccaattggtgtgctaattataaacttttgatctattcactgaggccaaggttttaagcacttctacagtgaaatgctataatgtcctttttgatattttctctgtgtgccttaaaatattctgtagttgttatttttcactgattcctataagctttcttcaaaattgtatcttattgcatatgaaccacacatgtaattttgggtataataatttatcttgctaagacattgtatacttattgtacagttttatacaacaacatatattacatattcacacaatctacctctttgtatgatgtagaatagtggctgtgaactgggagaaattttggcaatgactggagacattttgattgtcattactaggaggttcttactggcatctagtagacagaggccagggatgttgctaacatcctacaatacacaggacagttccccacaacaaagactttcagctaatagtgctgcttttgagaaatctcgatgtagatcaagttaaaacaagttaaatcttattgaaggcttcagaaatactcatcaaatgtactgctactttggactgaatttcattatttctaaaataaactaatattttactcttttagttttttttaaaatacagaaacgataaagtatttgttctgaaaatcagaaaactaagtctttgaaacagatggtacaaagaatacattgcaatttggccactagtattttctagatcctactcttaagtttctttaatatttttaccatataattttataattctataaattatacagtcatgtaatgtctgtgtttccaagccagattctgttaccgtaaggctgttcacaggagtctgggagattcagagaggctttcttaacaagaggattcaaggactctgagaaatgctatcctagtgtacattatctaactctttcactcatctttgttctcctcaaaattactgagaacattgtaccactagaaacatttgctagaaagtacaacttctagcaaaaaattagactaaaaaggaaataaaaatacgattttttggctaataaaataacctgaaatccaggaaaattgtgaagtcttaagaaacacaaatgtaaatccaatgagaccttgataaacaaaaattcaataagccaaaaccataattaaaacttttcttgacgaaacaacatattacaggatgggtcctggaatgtgtatatatacattcctataacttttgacttccagaatcatgttaaatggtagtaggtgtctctatttggttttgactctggtgcttttctggtgagttatagataccttgtatcatgttaaggatattctttattccagctttaaaagagtctttaataagggacaagtgtttggcatctattgacataatctagtggcttatattatttgacctagggacaaaagcattgattttgtatcattaaactctttatgtatttctattgtctataatgatgactgagaccaagatagcaaacagatcactatattttataaagatttccagtggtaagtatcgaaccaatttccagtggtaagtatcaaaccgaaaggtattttctaaggaaagcccttgtaaatcagaaatgtcataaatcagaatccctttcccaaaacattaactgagattttactgaatcacactaaagagaatgaccagtttggtttgtgaatgtcaggctgcaagagcacctttcgattgcagaccctactgggtttgaacagtaatatactgtgtaactggcagacaaggatacaaatgaagcttttaaaatatatcactttagaagctgaaattggggtgtgtgaaatttccctttttgtgaagtcagttctcatagctaactctattgttcctatagattccccacacctactaccaactcccctatagagtacaagccaggctgaagaaaatgctttgaggtgacccaaccctgcatggtttgtgctaaaaacagcaacccattctgaaggtgatagaaatgaaactgattgtgttgggaataatttactatactggcaatatttgattttgacacaactgtgaatgatgtaaaacatggagagagaacattaatcagactcttgccataagaattcaataaggttctagtacaatgaaagttacagatgaggagaaaactctgggttcttgttttgttttgttttccgtttcagttgggtatggcaaatatatttgaaatgcactgacatcttcaaatgcagattttttaaattgttgagtgtggcccaattgatagaaatagtttaccatgaatctttttttcttctatcacaacatgcttttttttcttttccccttaagatgttaatttatcatgcaaagattttttttcattaagtgcattaatgcttttgtttgtacaggaattttcaaatcaagaggactccccgtagttactaaatataaatccttatcgaatgacatgccaagatgatagctccattccacatgggaaaaggcaaattcagccgtattttgggattttaaccagggctccagcctttgggttgcacagtgtctctgatacatctcttttatgaaaatttcagattgactgtaaatggaacattttgtagaagaaactggcttctagcagttgagtagtgatgctgggaataaatttggtttccctgaatatggtttctcaaagcagtcacagcttctttagaagtcagaattggtaccatttcttatccttgtatttcagcattaactcatgtgcatgtttggaaaatgcttctgcactggtcatcatgcctgcagttttctcttccagctctcctagcctctgtcctctttcatcaagtgcaatccgtgcacgggtcagctctcccatcacccctccagcagcgcctttcatcccttctatactacctggtccaggaatgtgttgcgcaaggctgcgggatgcttttcctgccgaagcttccccaaagagctcttctctgtcaaatgtttgtccgcttccaccaaacagtcccttgagaaagcctctgttttgagcttctggtgtctctatgggagtaaacaaatctcctagcatgtcctgtagattatcacacatttcttggctgtatgttaaccgctgaatttcagtaggagagacgaggtataatgcctgtccttcattggtaaaacaaaatgttcgtgctatcctcatgtctgtcagtggcaaataattaacatccaacattgggcgaagactaggtaggctcattatcatgatatgtccgttagcacaaaagcatgccaagcaggcactgctacacatgaccaccacatttgcttgcagtataaaagatgtctccgtgatgttatgaacataaaggcaagtctgagaaggcagtgagaagactttggcttgtttttctgagcagattattgtatactgatgatctcctatttcttgggatgcagaagatgagttcattaccactttccttctccaagatttttcattttcatctatgttgtttggatccctccaaacttcatatggcggttgcattaatccacccattcggtccatacaggagaatgttagcacagctcctttcaatgagaggaatgtaccacttggcaataccatgactggctctgtaaacctttgttcatctgctaatggtaggtttaaggagatgattaacaccattcccagactggttccaacgaacagacaaggagagatggtagagtcatttttccgtgcaaaggagtccatgaagtatagtgctgtaattgcttctttagaatctttgtcaatactggagatactagagcttctagaacgattataggaattttctcggttttcttctgttgtaactggtaaagaaatctccatgcaggctgctgactgggcctttcgaaatggtggtcttccaggaccccagcgatttacttttgaaacatcggcactagaaagacgttttccagaactgcaactctgagaagttggacttgtgcagtgtccatttacatggtctgaggtaggagacttgcagcgctcaagttctaggggaactggactgtcattcagttcagttaaactctgataggaagtacggatccgtttcgttaaatcaggataaaagttagacaggccacgcatgcaaaagttgtctgcaatgaactgtttgttttttcgaggagaccgtggttgtcgctggtataagtcacttgatctatataggtcaatggtccccatgcttaacagtactgtcttctgtataaaatccaccacagccaacccattgcagttcccaaatgcaactattccatatgctgagcttacagcaagactagtaatctgttgtggaggttcaccatctacccacaccaattgaataacaagttctgcttgatatcctggaggcattcgcactggccgtgtcttcacattgaggcatggaatactgtcctttgttactccttcactagcaacagtgttagtgctcccagaaagactccttgaagaaggaagctgggctgagagatctggaaacggaggacttgtttctggttcaggggtaataatatcttcaacatcatactgaagtcgtacctctaatgacactatttctgttgtaatttcatgtctgctgaatttataaattatgacatatgcagagactcctgatacacagaatattctgctctctggacaccagtaaatcatctgaatggcaaatgggtcttcctctacaatttcacatgtttgttttccttctcctaccttctgtttttcaaacacttttgaagtttttagcttgtacagcatctgcagagttattgcagaagcatcccaaaattttattgatccatctgcatgaccagtaataataatttctggatatgtttgtgctccaaggttccaagctcctccactgattggccactccttattactgtatccttgttttttatgcttgactcctatagaatacagtactagaatcaaatccggaggacaatctgcaaagtatgctgtgcatgtaactggtgattcatgaatgtccatgggatatggattttcaaagattggaaaattgctttgtgtcagatcaactacaatgagatctttctccagaagtaccacgacagcatagggttcttgaaattcatttggatagggcgtttcacataaagttagaaattcaacaataggatgatccatttcaagtactgtaattgcttttccatgcatgatggttaaacttggtcttctacaagctttgtcataggacagcccaccagagaatattatgaatggttcgctgtttttgcaggtcttgtattctactttaagaattggtttacaagattcagattttcttccttctctttgactttttccatgtggaattgtggtctggaaagggcgacttgggcttttcaggttccataaagtcaaactaccatctgaatggctgcacatgaactgtttgccctcatgatgccaatcaattgaatgaatagcctcatcataataaactctcagttctgctcttttagatttcaagtcccagaatactacagtaccattttcataacctattagcagtttgccttcatctcttgggctatcgcttaaatgtacaactggacctggatgagtcttagtggatagttcaattgccttgttccacatgataacatatccagaaagaatgaaagattcaatatttacaatatgtgtatttcctctttctgttccaacataaagccatttactctggaaaggtagatgacagtaagtaattcgttcccggttaaatttaagagaatggagtatggctggccttttttgtctaaggttccacaaatgaagtgtatcatctgaacttgcactgaccaaggcaccctcattgatcaaaaattggagctgtaggacagctgcaccactttcatgttggcaatagcaatcaacaccaggtctcccgagtattcgtatagcacctgttctcgtcccaatagccaagattttctgaactggatcaaaggctaatgctgtgggctgatgaggaaaaccatgccgaactgtcttgcaaatctggaaatactccgaagtcaaagtttcctgaatttcctctctgagaacccctgcagtccccgccggatgtacggaaccacttccagccccaccaccactgttactgccactgctgctaccactgccaggggaggaggcagttaagccatccaaaacttttcggaaattaaacttcttcattttaaacacttcctcagacgcctctagccgcctgccagcccgggaagctgagggggccgaggtaggcgggctccggccgcttctctgggccctctggtcgcggcgcctggcgctctccgaggtcctaaccgagcagtc

SEQ ID NO: 8896 - RNA, 8620 nt, Homo sapiens
  source 1..8620: mol_type = other RNA
acagcactgcctggtcagaaattctcaaatgcttttgttctgtgagacatacagaataaataccattactatatcttacatcttgccttccctgaccactcagaactggggctggagcaccagccaaggcagacaaacaaggtttccttagttggccataaagcagtgataatcaactttggctggacattagaaccgccttggaggctttcgcaaatattggtgtctggttcccactccaaatgattttaatataattgggaatttaaaaatttcctgaggtgattcttatgtacagtcaaggttgagaatcactcctctagataaatgtgtaaatcaaagcatccatctgtgcatctgattccttaaagcctctttcacttcactgtggctcccatgtccttcctcaccacgatcttcttgcaccaaattggtacttcctcctccttttctaagacagaccttacctattctacatttcatgctttcagggctatgttgtctgcaaatacacacactaaacttgttatgttgacaaccatgttccctggaatggtgcatactagaggtactgctcaaaccaagtacaccacaagtatttctggcacccaggacagtgtgcatgtgaaatagtacctagccaaaaatggagttgcatgacagaggacagaggtgaagaagctgtgaaagccaccacgtttctcctgacacagataccaagacctgatatgaatgttttgacttcttttgcattgccctgtgtgagccaacatggtcaagttacaattcttttttctcatagcagcaggttgtaatcacacagatatactcccagtttgacccaatgatcctaagccaaggagaggatttttagcttacttttctagattggcttcatttttcccttctgcttgaatataagaatctattttaatcttcttcaaccaatgttaggcctaatctgattcttttttctctcaaagtcatggtgatcccttcatgtagataaagtatagatgatgcctttaaaactggtacatgggtcacataaaaagggactccaacagtaaaccttttccttcagatccctagaaactttgagggaaaggagttggattttgatttatttatttgagaatcactttcaaaagatctgagaaaattgtctttgtgactgaatcactggaaaacatctcattcagttctgtcactgtcctttcagagttccagttagacaatgatcttgacaatgattggggccctaaagtctggggctcagtgaagtgtaagaagcaaagtcagtagtactgcttttgtaggtgattaaaacaaatgaggaatcaatcattcctccctccaaactccaagactaatggatgatttcaaggtagggactattgctcacgttattatcagggaaacaaatacctctagcttctcacagatgaataaatgaaaaggcccattttctactgtaacactaaaaaggccttatcttccaaggaaatcatagggagacaaggtcaacttgttgggactgtggtttgcaagccttatcttctgatgtcgctttagcagatagaatgtaattttgatggtaactaaggctcagagtcactttctgtatcattgtccaagttattaggagtatttttcttatgttccgaaatagaagaaagatagtaaagatgagactatgcaaaggattacatggatcaacagtacttattttccaaagatgaggataagatgatgatggtagtggtggcgatggtgtgtgtgtgtgtgcgtgcgtgctaaggtcagtgcaacagaacagaattgttcaaagagaaaaatcacatccacattagattcttcttattgctatcatctctttgaattataaaaataattttgatacagtaaaacctcattaatttggattccactaaccaggagtttgtgagatgaagttacccttacgttaaggaagggcttataaaagcaattttgaaagacacgttttaactacttcaaagagccttttcttttcaagcatttgagaagcacctgtttacttccaattggtgtgctaattataaacttttgatctattcactgaggccaaggttttaagcacttctacagtgaaatgctataatgtcctttttgatattttctctgtgtgccttaaaatattctgtagttgttatttttcactgattcctataagctttcttcaaaattgtatcttattgcatatgaaccacacatgtaattttgggtataataatttatcttgctaagacattgtatacttattgtacagttttatacaacaacatatattacatattcacacaatctacctctttgtatgatgtagaatagtggctgtgaactgggagaaattttggcaatgactggagacattttgattgtcattactaggaggttcttactggcatctagtagacagaggccagggatgttgctaacatcctacaatacacaggacagttccccacaacaaagactttcagctaatagtgctgcttttgagaaatctcgatgtagatcaagttaaaacaagttaaatcttattgaaggcttcagaaatactcatcaaatgtactgctactttggactgaatttcattatttctaaaataaactaatattttactcttttagttttttttaaaatacagaaacgataaagtatttgttctgaaaatcagaaaactaagtctttgaaacagatggtacaaagaatacattgcaatttggccactagtattttctagatcctactcttaagtttctttaatatttttaccatataattttataattctataaattatacagtcatgtaatgtctgtgtttccaagccagattctgttaccgtaaggctgttcacaggagtctgggagattcagagaggctttcttaacaagaggattcaaggactctgagaaatgctatcctagtgtacattatctaactctttcactcatctttgttctcctcaaaattactgagaacattgtaccactagaaacatttgctagaaagtacaacttctagcaaaaaattagactaaaaaggaaataaaaatacgattttttggctaataaaataacctgaaatccaggaaaattgtgaagtcttaagaaacacaaatgtaaatccaatgagaccttgataaacaaaaattcaataagccaaaaccataattaaaacttttcttgacgaaacaacatattacaggatgggtcctggaatgtgtatatatacattcctataacttttgacttccagaatcatgttaaatggtagtaggtgtctctatttggttttgactctggtgcttttctggtgagttatagataccttgtatcatgttaaggatattctttattccagctttaaaagagtctttaataagggacaagtgtttggcatctattgacataatctagtggcttatattatttgacctagggacaaaagcattgattttgtatcattaaactctttatgtatttctattgtctataatgatgactgagaccaagatagcaaacagatcactatattttataaagatttccagtggtaagtatcgaaccaatttccagtggtaagtatcaaaccgaaaggtattttctaaggaaagcccttgtaaatcagaaatgtcataaatcagaatccctttcccaaaacattaactgagattttactgaatcacactaaagagaatgaccagtttggtttgtgaatgtcaggctgcaagagcacctttcgattgcagaccctactgggtttgaacagtaatatactgtgtaactggcagacaaggatacaaatgaagcttttaaaatatatcactttagaagctgaaattggggtgtgtgaaatttccctttttgtgaagtcagttctcatagctaactctattgttcctatagattccccacacctactaccaactcccctatagagtacaagccaggctgaagaaaatgctttgaggtgacccaaccctgcatggtttgtgctaaaaacagcaacccattctgaaggtgatagaaatgaaactgattgtgttgggaataatttactatactggcaatatttgattttgacacaactgtgaatgatgtaaaacatggagagagaacattaatcagactcttgccataagaattcaataaggttctagtacaatgaaagttacagatgaggagaaaactctgggttcttgttttgttttgttttccgtttcagttgggtatggcaaatatatttgaaatgcactgacatcttcaaatgcagattttttaaattgttgagtgtggcccaattgatagaaatagtttaccatgaatctttttttcttctatcacaacatgcttttttttcttttccccttaagatgttaatttatcatgcaaagattttttttcattaagtgcattaatgcttttgtttgtacaggaattttcaaatcaagaggactccccgtagttactaaatataaatccttatcgaatgacatgccaagatgatagctccattccacatgggaaaaggcaaattcagccgtattttgggattttaaccagggctccagcctttgggttgcacagtgtctctgatacatctcttttatgaaaatttcagattgactgtaaatggaacattttgtagaagaaactggcttctagcagttgagtagtgatgctgggaataaatttggtttccctgaatatggtttctcaaagcagtcacagcttctttagaagtcagaattggtaccatttcttatccttgtatttcagcattaactcatgtgcatgtttggaaaatgcttctgcactggtcatcatgcctgcagttttctcttccagctctcctagcctctgtcctctttcatcaagtgcaatccgtgcacgggtcagctctcccatcacccctccagcagcgcctttcatcccttctatactacctggtccaggaatgtgttgcgcaaggctgcgggatgcttttcctgccgaagcttccccaaagagctcttctctgtcaaatgtttgtccgcttccaccaaacagtcccttgagaaagcctctgttttgagcttctggtgtctctatgggagtaaacaaatctcctagcatgtcctgtagattatcacacatttcttggctgtatgttaaccgctgaatttcagtaggagagacgaggtataatgcctgtccttcattggtaaaacaaaatgttcgtgctatcctcatgtctgtcagtggcaaataattaacatccaacattgggcgaagactaggtaggctcattatcatgatatgtccgttagcacaaaagcatgccaagcaggcactgctacacatgaccaccacatttgcttgcagtataaaagatgtctccgtgatgttatgaacataaaggcaagtctgagaaggcagtgagaagactttggcttgtttttctgagcagattattgtatactgatgatctcctatttcttgggatgcagaagatgagttcattaccactttccttctccaagatttttcattttcatctatgttgtttggatccctccaaacttcatatggcggttgcattaatccacccattcggtccatacaggagaatgttagcacagctcctttcaatgagaggaatgtaccacttggcaataccatgactggctctgtaaacctttgttcatctgctaatggtaggtttaaggagatgattaacaccattcccagactggttccaacgaacagacaaggagagatggtagagtcatttttccgtgcaaaggagtccatgaagtatagtgctgtaattgcttctttagaatctttgtcaatactggagatactagagcttctagaacgattataggaattttctcggttttcttctgttgtaactggtaaagaaatctccatgcaggctgctgactgggcctttcgaaatggtggtcttccaggaccccagcgatttacttttgaaacatcggcactagaaagacgttttccagaactgcaactctgagaagttggacttgtgcagtgtccatttacatggtctgaggtaggagacttgcagcgctcaagttctaggggaactggactgtcattcagttcagttaaactctgataggaagtacggatccgtttcgttaaatcaggataaaagttagacaggccacgcatgcaaaagttgtctgcaatgaactgtttgttttttcgaggagaccgtggttgtcgctggtataagtcacttgatctatataggtcaatggtccccatgcttaacagtactgtcttctgtataaaatccaccacagccaacccattgcagttcccaaatgcaactattccatatgctgagcttacagcaagactagtaatctgttgtggaggttcaccatctacccacaccaattgaataacaagttctgcttgatatcctggaggcattcgcactggccgtgtcttcacattgaggcatggaatactgtcctttgttactccttcactagcaacagtgttagtgctcccagaaagactccttgaagaaggaagctgggctgagagatctggaaacggaggacttgtttctggttcaggggtaataatatcttcaacatcatactgaagtcgtacctctaatgacactatttctgttgtaatttcatgtctgctgaatttataaattatgacatatgcagagactcctgatacacagaatattctgctctctggacaccagtaaatcatctgaatggcaaatgggtcttcctctacaatttcacatgtttgttttccttctcctaccttctgtttttcaaacacttttgaagtttttagcttgtacagcatctgcagagttattgcagaagcatcccaaaattttattgatccatctgcatgaccagtaataataatttctggatatgtttgtgctccaaggttccaagctcctccactgattggccactccttattactgtatccttgttttttatgcttgactcctatagaatacagtactagaatcaaatccggaggacaatctgcaaagtatgctgtgcatgtaactggtgattcatgaatgtccatgggatatggattttcaaagattggaaaattgctttgtgtcagatcaactacaatgagatctttctccagaagtaccacgacagcatagggttcttgaaattctgatattagaacctgaaatgccagcattgctgtactacatctgtgttatttccagtttctcaagtaggtacagttgcagaacctgttccagcacttgtagctcacagcgttataccacagtagacatcatttggatagggcgtttcacataaagttagaaattcaacaataggatgatccatttcaagtactgtaattgcttttccatgcatgatggttaaacttggtcttctacaagctttgtcataggacagcccaccagagaatattatgaatggttcgctgtttttgcaggtcttgtattctactttaagaattggtttacaagattcagattttcttccttctctttgactttttccatgtggaattgtggtctggaaagggcgacttgggcttttcaggttccataaagtcaaactaccatctgaatggctgcacatgaactgtttgccctcatgatgccaatcaattgaatgaatagcctcatcataataaactctcagttctgctcttttagatttcaagtcccagaatactacagtaccattttcataacctattagcagtttgccttcatctcttgggctatcgcttaaatgtacaactggacctggatgagtcttagtggatagttcaattgccttgttccacatgataacatatccagaaagaatgaaagattcaatatttacaatatgtgtatttcctctttctgttccaacataaagccatttactctggaaaggtagatgacagtaagtaattcgttcccggttaaatttaagagaatggagtatggctggccttttttgtctaaggttccacaaatgaagtgtatcatctgaacttgcactgaccaaggcaccctcattgatcaaaaattggagctgtaggacagctgcaccactttcatgttggcaatagcaatcaacaccaggtctcccgagtattcgtatagcacctgttctcgtcccaatagccaagattttctgaactggatcaaaggctaatgctgtgggctgatgaggaaaaccatgccgaactgtcttgcaaatctggaaatactccgaagtcaaagtttcctgaatttcctctctgagaacccctgcagtccccgccggatgtacggaaccacttccagccccaccaccactgttactgccactgctgctaccactgccaggggaggaggcagttaagccatccaaaacttttcggaaattaaacttcttcattttaaacacttcctcagacgcctctagccgcctgccagcccgggaagctgagggggccgaggtaggcgggctccggccgcttctctgggccctctggtcgcggcgcctggcgctctccgaggtcctaaccgagcagtc

SEQ ID NO: 8897 - RNA, 30 nt, Homo sapiens
  source 1..30: mol_type = other RNA
acagcaggcacagacaggcagtcacatgac

SEQ ID NO: 8898 - RNA, 7816 nt, Homo sapiens
  source 1..7816: mol_type = other RNA
acagcaggcacagacaggcagtcacatgacaacccagcctgaatgacaaccagccattgaaagaaagcagccctcacaccatagcatctacaccaagagctacaaccaaaatgaggggctcgggggcctggggttttaatctgttggtttaatacttaactcatgtattattttattttgattcaagtattaaaacccaccaaaagtaaagtgagtggtgcctatgaaatataataaaacccatttctgaaaatgttcctgtgcattctatagttctcttttcctaattgttgtcagcaaatcactacccttgacctttattgtacacagctttgcagcaccctatattgatataaaaactcaatataacaaaacaatataacttcagtctgatgcttaacaaagaataaattattctaagaattcttgtccataaactaagtatggttttctatgtcatgattttttttttttttttttttttttggaaggggatagggtggaaagacagagaaaagaaaagggagaaaaagagtattccaaaggatcaagtgctttgagttaactctgccagtctgggttaactctgccagtctgggtctgggcaaaacacagtgaaaagactactatttccaactagtgttcaactatattaaaataatagtttctcctcttttgacatatggaaagttgaaatttttgatacttccacgcgtcatggtatacataaatttatgactgcgtcattctttaattaagaaggtgcttatgctacagttctaggagtagaatttacaaggccaacacattcacttgcaacctatgcttccatcactataaactttcaagatcttgagatgttcaggcaattcatttatcttcagaagcataaggaaagtggttaatgcacttgaaatgtatattttgacacatcttttgagaaaatatccaaacttcagtttatgcactgttaactggagtgaaatgataagggatggcttttgtctatgaatactttaaatacttaagggtaaaaggtgggaagatggataaaattagaaatgtgtcaacttttatttagttcattaacatgttttagcttcagtatttgaaattaattttcatctttcttagattctggtcaagcttaaaaaatgtaacacaaggctactcaaaacttttttcacatttaacaattaaacactttatgtatgtattcttaactaaagcaaactatttttcattcagctattttatttttaaaatgaaagtctcagtcttaaagctaagatcccagtgagtttcaaattttctgacaatgatattttaaccaaacctgacattatagtttctttaattaaaaaactgaatgatggggcaaaactacaaagcacaaatatgattaaagttaaatttctctcatttaaacaatcttgtcttatggcaatatgtcatctgctaaaattcatctctgcttctgcaagatacattgcacgatgcagatttttgccttaaataaaagtcccattactagcaaataaagtcctaaacaatacttacaaaatgtagaatataaacaggaagacaatataaaaattactcacagaatatcgacatcgttctacccaatcttaaatgccttgtaccacctgttgcaaatgctgcctatgagagttcacgtatggaattattctactggaccctgcaaggctcaggagagtgcttgacagctcccagaatgagacaatgacctagccagaacattaaggagactacacccgtccttcagactccaaagggaaagctaggacggcagcagagtcatcctaaggtgaggcactccaggataacattttcaatatttttccttaaaacataaagttaacaccttttttgttaaacattttttactcaattttcaaaaaaaatgcttgaaagaatgttttgtatgtattttaaagtcattaaatgaggcacatttaaaaatttttctcttctgggaaagggtaatataaaggataatattgctcttccaggataaacttttgagtgggacaaataatgcatataggggagtgggtttgaatctaaactcatttttaataaatttggaataggattggccattatggtttattgaataatactctttttttcaaaattataaatctttagataataccagaacatggaaatatttgtatgaataatcctatattaaaaaagaataacatcagatagtttatgtatgtaaaaaaatatacaactgtgatcatgcagaattttaagtaatataagtggattagagttcaatatttactgggacttttgtgaaaatatctaagttttggctaactaaataacttaacgaaggagtgtgaacagtgttcacagggtcgacgctgaccttttccaccacagggagtgtgcagatctggtaggaaatatgcacaatcttaaaagtataagtgaaactagaaagagagctgaatatttctataacttcttgatctcacaactttgatcatccagggatataactgtcattttgtttcctatttctgaagttacatttgtcatttgttattgttacaaaatgaaaacaatgctaagtaaatatccctataagggaattatataatctccttatcaagttatccaaacacttcaacccacaaaaatgaggcctgtaatttcttaagagtccaaagaatgtccttatttcaatgcagatgttgggttttcctcaatagtataaggttagcagatttccactggaaacgcctatgttgcattattctgcttgcctaggagtagctcattatgatttaaatctttacacactgggctatagaaatagaataaatattgactaagtgcttttattatacataaattaacagtcctctttcttcagagatttgaattatctcttaaaatttacatatttatgtatttttaaaacaaatttctcattggttttaagaaaaataaggctcttttctccttgaatcagggtctcccattctcctaaaattcacattttagacataagttaaagaaaagccatcatttttttcaagtctgattttaaagtattaatgtaaaattatctagatcaaaaatccatttcaaaaaacttttgaaatgacagtttctgttttattctcacatcttgctttttactaaatccctttccaaaaatgtacaacatatatgggcaatgtatgaaaacaacattgggaaattaattttctgtttaaatgattttcaatccaggaagtcacatatatatagtcagaggataaaaaacaaacaaacaaacaaaaaacaaaaacaaaaacaaaaaaacactaaccttcaatgatgaaaattaacaaaatttaagacaatttaagacaatctacctttagtggtaattttattctgtaattcaataatttaattttgacacttgatatgccaggacgtgattaattattatgctgcatttattcattcatttgctcaatgacaccttcattcaatcaatatttagttagtgtctcctatcagtgctatgtcccctggtggtaggacagggaacaaacaatgtctcctggtctcaagaggcttacagtttgctgcaactcttagcatgtgtgatgagttgttcatgtcaattttcaccttccaaaaacatctcttaaatccgttcatttttatcaaattccaacaactcatcccagcccaagctaccattatctatgcagaccacaatagatgtagaaagcaatagctttctagtaactccccagtccagtttcgccctcttccaatccattctccacaaggcaaccaaaggaatcagtaaagaattcaaatcttatcatgtgactctccagcttaaaaaacttctcatcattcttaatatcaaaatcctcatctttagagtgcctttctctttttgctccagtcacactggacttaattaccctccttaaattcatcaggctcaatcctgcctcagaacattaacacaaaccttctctgaccatccaatgtaaagtaccccctacctgtgtcctctatcccagacactctatgtcaactcatcactggctttattttcttcctagcctgtaatcagcatctgctaggttttcctatttatttgtatgtttgctttattgggaaagagccttcataagaataggtaccatgaattccttgctaatcattttatccttagtgattaggacagtgcctggtacataacaagtgttcagaaagtaattgttgggaaatgttcagatgattaagagcacagcactgacacttagcacctggctaagttactcactctcttttgagcctcaattctttatctctaaaatggagaatgtaaataatgtgctcagtgaactataaatactcaataactattagccattatggtgatgatcctcctcattaagatcatcattgagtttgagttgtggttgcaagtagcattccccctagtcattatacctgcttaaattcacgaaggccagctttcagtctcaatgatgatcttaatgatgagaacttcctgtcttgtttcttgagagttctgaatgagtaacagaagctagtgactcaatcatagctgtgtgtagcccataattttgctaccttgaacttaagtgctccgcaccctcaccaccagctactacccagccaccatcctctcttgcctggaccatggtcagagtttccaatctggtctcccttcttccatgctagccatccccgctcccttcacgcatccaccccataccacttattatgcacaatccagcagccagggcaatctttctaaaccatcaatccaatcatgtcacaacctgttggaacactccaatcattttcagttatccttgtaataaaatccaaaccattgggtagggactgataaggcccccatctactggtacctctgattttatctcctttctcccccactgttcctatgttacagccacagacttcctgttggatcccatctccagggtttttatacttactgttccctctacctggaatattcttcagcaaaatcttctgcacagctcatcatctcagtctctgctcaagtggtacttccttccaatcacccaaatctaaagacccctcccctatcactttctaactcaatgccccattttattttcttcagagcatttactatctgacatttattactagtctatttgcttgttagctccatagaacagtaactttgtcatttcctcttttttaaaatgatctaaatggatgaaactaccctttcctagaatttcttcatctaaataattccatttatttcaagggtcatttccactctcacctgcccccaactaccctccataccataccttggttatacacagcacacagagcgggagtattcatggcacttggttaatattataactgtgcatatttattttccatttgttgtaatcaagtactcataaggaagctacaagggcagtgattttgtaaagaattatcctgagtctggaggagaggagatgagccaataaccaagagctcaccaagccttcaaagcttcttccttccctacagagagcatcctataccttccaatgggcttattttcaggactcacagagccagactaatgccacactccaacagcagtagctactccagagtcttcagtgtctctgctgctaacacccaggaacatgtcaatgctgagatgcctggaattcatcttcataagtcctctgtgggatgaggttggcttggacaactccaggcatctctgggattcttgcctttatttgtggttgaaagcataggctctggagctcaacagcctgggttcaaatttctgctttgccaccaactagctgtgtgactttggtaagttggttatcctcgccaagactaaatgttctcatcatctttataccaggacaagctttccgcagtaaggacgaaccagtatcccttcgagccgcctttcatgatgccaatgttgctgatggtgagccaccccttgcgaatcacagaacttagctcgtacaatttgccttgaaggcggaagattggttccctgatttccaactgtggttttcttgtgaacctgactgctcctctgctgagcatttgcgaagccaatgaagtcttcatggttggtgttgatgtaagagacttgaatgtcaatcaatagcaatacctggtcctttgtcttcccttctcgctcacgaatgtggttagcaacaatcctttccgtttcctcgcagagtctggggaagtttgccagttttttggtacacttcttcacagtgttgattaattcttgtattaccagatccacactcttcaaggaaggccctttcaactttacaatctgtttcttgactatcgcttcaaatgccatgtctggagtaaacaaccctgtcctgataccatgtatgtttttgattgcatagcttatttctcttcgcaattctttctcattgaactccatctttactatctcaaaaggaaagcgttcatgaaaaatacgattgattttagcaccacctgagagttccagggtatctacttgatcccctgacccttcaattctcttctcaaagtccacagcaaattgctgaaccatctgcagcaatgctttggtcttccttgttgggtcttctggtttgaaatttttgtaggcttctacttcatgttctatggagagcaactgtccctgtagtttgttcctgaagtttggtagggtatcccgaatgtggttggtaagttgctgattaaggaccttctgcaggtgtggggttcccattcggtcagcgatatgtctgtaagccgggtgggaaaggaaaaacttcctctctgccagcatggctgcctttatgtccttcttcccatctatgtccttctggcttctgtttaccacccccacgtaacccctgcgaagaggcaacagtttgttctctagaacatccctggcatccgttccttcatccataaggtccagtttggtgataactccaatggttctcagaccttgaggatcaacttctttagctagcttcagcgcatctgagtttgcaagatcagtgttggctggagtaacagctaaaatcagacagttctccctcgtgatgaactgcataatcatttctctgatctgatactcgatatctggtggctgatctcccacaggcactttagttattccaggtagatcaataagggttagatttaacacgtgtggggaatagactcgtaaattaatgggtatggaggaaatgcctttattcattccagtcacgcgatctgtttctgcttcaatctcaaggcgaacttcatcaaaatctgtaaatttctttcctttgcaatgtagaaactcggcatattctgctttagaagtaacaagctgcagcacaagaggtcgtcttgttacaatgcccgaccctcgagggagaaagtccctgcccacgaagttctcgagcaccgagctcttgccggcgctctggccgcccaccacggcgatctgcggcagctccagcaggcagctctgtcccagcgccgaaaacgcgtcctgcagacggttcaccagcgggatcagctcctccatctcccggttccccatcttgcccgaggggccggcgaccagctggtccctgctcgcctctacgacctgacagggagtaggggccgcgctgccctggctgctgctgctgcgccgggctcagccagccaggtcctggcgcagacgtcggagcccgccgccagcccgccgcttggctctgac

SEQ ID NO: 8899 - RNA, 40 nt, Homo sapiens
  source 1..40: mol_type = other RNA
acaggagtgggggtgggacataaggaggatagggaacaca

SEQ ID NO: 8900 - RNA, 61 nt, Homo sapiens
  source 1..61: mol_type = other RNA
acaggagtgggggtgggacatgaatgctgcaatgttctgcagcctcaggccccagacgcca

SEQ ID NO: 8901 - RNA, 67 nt, Homo sapiens
  source 1..67: mol_type = other RNA
acaggcacgactggtttggcaattcagtaaaaatgctcaaaccggctgtgcctgtggacgcagccca

SEQ ID NO: 8902 - RNA, 2511 nt, Homo sapiens
  source 1..2511: mol_type = other RNA
acagggccgcagatggagactgctcaaggtcaaaggggtctccagctgggaccctgcacctggttcgtagcccctctgcagacgcacagtgcctcacgcctgctgcaacctggaaccttgaggccttcatgtcagtgcaggacaagagtcatgtctgtccatagattggggctggaaaggactttctgccactggagcttcgatagtgagcatgcatccccgccaacagctgtgtctccctttgaaccaagtctggttcctccaagcaagcggtcgttcattccaaagagggcctgatcccagacagttaactccaagcttgactgcctcagctgagctggggttacgccactgaagacaaatgagtgtttccactgggggcaagcctgcttcctcaggactggcgacttcagtctcagtttttgttggtctggcagagtgagacagcccttaacaaatgagttcaaggtgccatctggccgcacaggtaaattcttggctcctagcactaccaaacaaagttgaccatgaagtgatggctgatctgtcccttcttgagcctcttggagttttctgggccgtgaagggagaaccagcttagcccggactgtgagctctccattactctgaggaacgctgtcttcgtatttctccgccttggcccggagcggatgccagcggaaggactgtgttgtgctgtcttcaaagtcccacgtggccagaggaatgatcacttctccaagaaacactctccgggccagcgtgcccagatgccacaccgagacctgcagctgccgggtcaccagctgggcaggggccacctgatacttcaaggtctcctgaaaggtcgggtccacggtgttcctttggactccagtcttgcgctttccctgggaggatctgtcgggcaacaggtaggtcttcacatacggattgcactttttcttcttttcttctccataggcaaggttcttacaggccttgatgcatatttctaaagaatgggttttgaagcaataatgaatggcaaattctatttctccagtgacattagcattgtcaaaattgcccatctctgtacaggtgctgtcaatgctaattaaacttccgtgtctaaaacctccagagaatatggtactgggtgccggactggatgggagattctgttgcttcaaaatagggttagtagagcatttgggatcctcttgattgagaggtttcagaatatctggtgcactgaccttcctgccaggactgcggctgcactggctctcgctgacaggaggtggagtaggaggaaccacagaaattttgctcagcttctgataagattgcaagagctgccctccaactgtctcatgtttgcctccagttggaaatttcttggctcgttcctcatagaaccattctccagtttttattttgacattcctgtcctcgaagcacaccgtgcacttccaggcatgggtccccctcaggaacactcggcactgggcacacacgcggtggctgcagccccggcacacggcgccccggtgcagcaggaaccccagcacctgctggcagcgcgcacagcacttctctttgtgctcccagtccgtgttcttcgctcctttccaccggagatgctgcaggtgtgttttcagtttccgtgtcctctcctcctctgtgttttgaaccgcctggtctcggtacaggacctggagaatggcctcgcgttctaactccttgagagcactcagatctatttcttgggccatttcttctccgttttcgttgacccaggttggaagagcttcactgcatggaccaagcgctcacgccctgcagatgagcggcggaggccagctgcagccagccttgtttaaagagctccctctcctatttcactggcaactgttttgcttgtggttcttttttcctttttaactgtgtcatactccttagaagaagaaagcctcaagaagttctgcgtttgtcggagttacggctcgcagagcctcgtgctacccggggggtgttttcaccgggttctgcagcagctgctgacatccatctaagacaaaagcatatctcttttctgaggtttcaccagagattgttataaattatccacagctgcaagcagataatttctgcaaagcagaagtaattttcaagccaaggaaatttagaaatagcaataaaaagagtatcagtgactcatagaagctaaccttccatttaagatgtttccaggtcagcaggaaccatcatgaaaagctcagcccgttcaatacctggctgggctggtacctgactatgccagcaggggcaacgcctcttccctccttagatccaggttccagatgaacaggcagaactggcatccctcagtgccccaaggctctgagtctctgagagaggacaaagttgaacaggcgctttctctgaaagatcactgcaattcaccgctgattccgagtattctttctcattcggggagccttcgcatctgcttcaagagaagag

SEQ ID NO: 8903 - RNA, 2103 nt, Homo sapiens
  source 1..2103: mol_type = other RNA
acagggccgcagatggagactgctcaaggtcaaaggggtctccagctgggaccctgcacctggttcgtagcccctctgcagacgcacagtgcctcacgcctgctgcaacctggaaccttgaggccttcatgtcagtgcaggacaagagtcatgtctgtccatagattggggctggaaaggactttctgccactggagcttcgatagtgagcatgcatccccgccaacagctgtgtctccctttgaaccaagtctggttcctccaagcaagcggtcgttcattccaaagagggcctgatcccagacagttaactccaagcttgactgcctcagctgagctggggttacgccactgaagacaaatgagtgtttccactgggggcaagcctgcttcctcaggactggcgacttcagtctcagtttttgttggtctggcagagtgagacagcccttaacaaatgagttcaaggtgccatctggccgcacaggtaaattcttggctcctagcactaccaaacaaagttgaccatgaagtgatggctgatctgtcccttcttgagcctcttggagttttctgggccgtgaagggagaaccagcttagcccggactgtgagctctccattactctgaggaacgctgtcttcgtatttctccgccttggcccggagcggatgccagcggaaggactgtgttgtgctgtcttcaaagtcccacgtggccagaggaatgatcacttctccaagaaacactctccgggccagcgtgcccagatgccacaccgagacctgcagctgccgggtcaccagctgggcaggggccacctgatacttcaaggtctcctgaaaggtcgggtccacggtgttcctttggactccagtcttgcgctttccctgggaggatctgtcgggcaacaggtaggtcttcacatacggattgcactttttcttcttttcttctccataggcaaggttcttacaggccttgatgcatatttctaaagaatgggttttgaagcaataatgaatggcaaattctatttctccagtgacattagcattgtcaaaattgcccatctctgtacaggtgctgtcaatgctaattaaacttccgtgtctaaaacctccagagaatatggtactgggtgccggactggatgggagattctgttgcttcaaaatagggttagtagagcatttgggatcctcttgattgagaggtttcagaatatctggtgcactgaccttcctgccaggactgcggctgcactggctctcgctgacaggaggtggagtaggaggaaccacagaaattttgctcagcttctgataagattgcaagagctgccctccaactgtctcatgtttgcctccagttggaaatttcttggctcgttcctcatagaaccattctccagtttttattttgacattcctgtcctcgaagcacaccgtgcacttccaggcatgggtccccctcaggaacactcggcactgggcacacacgcggtggctgcagccccggcacacggcgccccggtgcagcaggaaccccagcacctgctggcagcgcgcacagcacttctctttgtgctcccagtccgtgttcttcgctcctttccaccggagatgctgcaggtgtgttttcagtttccgtgtcctctcctcctctgtgttttgaaccgcctggtctcggtacaggacctggagaatggcctcgcgttctaactccttgagagcactcagatctatttcttgggccatttcttctccgttttcgttgacccaggttggaagagcttcactgcatggaccaagcgctcacgcccttccatttaagatgtttccaggtcagcaggaaccatcatgaaaagctcagcccgttcaatacctgactatgccagcaggggcaacgcctcttccctccttagatccaggttccagatgaacaggcagaactggcatccctcagtgccccaaggctctgagtctctgagagaggacaaagttgaacaggcgctttctctgaaagatcactgcaattcaccgctgattccgagtattctttctcattcggggagccttcgcatctgcttcaagagaagag

SEQ ID NO: 8904 - RNA, 2198 nt, Homo sapiens
  source 1..2198: mol_type = other RNA
acagggccgcagatggagactgctcaaggtcaaaggggtctccagctgggaccctgcacctggttcgtagcccctctgcagacgcacagtgcctcacgcctgctgcaacctggaaccttgaggccttcatgtcagtgcaggacaagagtcatgtctgtccatagattggggctggaaaggactttctgccactggagcttcgatagtgagcatgcatccccgccaacagctgtgtctccctttgaaccaagtctggttcctccaagcaagcggtcgttcattccaaagagggcctgatcccagacagttaactccaagcttgactgcctcagctgagctggggttacgccactgaagacaaatgagtgtttccactgggggcaagcctgcttcctcaggactggcgacttcagtctcagtttttgttggtctggcagagtgagacagcccttaacaaatgagttcaaggtgccatctggccgcacaggtaaattcttggctcctagcactaccaaacaaagttgaccatgaagtgatggctgatctgtcccttcttgagcctcttggagttttctgggccgtgaagggagaaccagcttagcccggactgtgagctctccattactctgaggaacgctgtcttcgtatttctccgccttggcccggagcggatgccagcggaaggactgtgttgtgctgtcttcaaagtcccacgtggccagaggaatgatcacttctccaagaaacactctccgggccagcgtgcccagatgccacaccgagacctgcagctgccgggtcaccagctgggcaggggccacctgatacttcaaggtctcctgaaaggtcgggtccacggtgttcctttggactccagtcttgcgctttccctgggaggatctgtcgggcaacaggtaggtcttcacatacggattgcactttttcttcttttcttctccataggcaaggttcttacaggccttgatgcatatttctaaagaatgggttttgaagcaataatgaatggcaaattctatttctccagtgacattagcattgtcaaaattgcccatctctgtacaggtgctgtcaatgctaattaaacttccgtgtctaaaacctccagagaatatggtactgggtgccggactggatgggagattctgttgcttcaaaatagggttagtagagcatttgggatcctcttgattgagaggtttcagaatatctggtgcactgaccttcctgccaggactgcggctgcactggctctcgctgacaggaggtggagtaggaggaaccacagaaattttgctcagcttctgataagattgcaagagctgccctccaactgtctcatgtttgcctccagttggaaatttcttggctcgttcctcatagaaccattctccagtttttattttgacattcctgtcctcgaagcacaccgtgcacttccaggcatgggtccccctcaggaacactcggcactgggcacacacgcggtggctgcagccccggcacacggcgccccggtgcagcaggaaccccagcacctgctggcagcgcgcacagcacttctctttgtgctcccagtccgtgttcttcgctcctttccaccggagatgctgcaggtgtgttttcagtttccttccatttaagatgtttccaggtcagcaggaaccatcatgaaaagctcagcccgttcaatacctggctgggctggtacctgactatgccagcaggggcaacgcctcttccctccttagatccaggttccagatgaacaggcagaactggcatccctcagtgccccaaggctctgagtctctggaaaacttaactccccaaagggaagtttcgttcagatagctaaagcatgccaatcccagtccccaagggaactgcaacaacgtctcaccgggcgcactgccttcagcagtcactttcgagtttgttgccaggtgtccgagcgggtttgaacgtccgcgtcaatccacacagtacaaaccggaggaggggccgggaccacgcttcccctccaggactgccttttgtacgtgtgttttgtttctgttgctaaggtttagggagctgcccggctaccctcacggattcccatggaaactaccacctcccagaggacaggaggagaggcgaattcagggtccacccacgggccccgcccagggatgggg

SEQ ID NO: 8905 - RNA, 1435 nt, Homo sapiens
  source 1..1435: mol_type = other RNA
acagggccgcagatggagactgctcaaggtcaaaggggtctccagctgggaccctgcacctggttcgtagcccctctgcagacgcacagtgcctcacgcctgctgcaacctggaaccttgaggccttcatgtcagtgcaggacaagagtcatgtctgtccatagattggggctggaaaggactttctgccactggagcttcgatagtgagcatgcatccccgccaacagctgtgtctccctttgaaccaagtctggttcctccaagcaagcggtcgttcattccaaagagggcctgatcccagacagttaactccaagcttgactgcctcagctgagctggggttacgccactgaagacaaatgagtgtttccactgggggcaagcctgcttcctcaggactggcgacttcagtctcagtttttgttggtctggcagagtgagacagcccttaacaaatgagttcaaggtgccatctggccgcacaggtaaattcttggctcctagcactaccaaacaaagttgaccatgaagtgatggctgatctgtcccttcttgagcctcttggagttttctgggccgtgaagggagaaccagcttagcccggactgtgagctctccattactctgaggaacgctgtcttcgtatttctccgccttggcccggagcggatgccagcggaaggactgtgttgtgctgtcttcaaagtcccacgtggccagaggaatgatcacttctccaagaaacactctccgggccagcgtgcccagatgccacaccgagacctgcagctgccgggtcaccagctgggcaggggccacctgatacttcaaggtctcctgaaaggtcgggtccacggtgttcctttggactccagtcttgcgctttccctgggaggatctgtcgggcaacaggtaggtcttcacatacggattgcactttttcttcttttcttctccataggcaaggttcttacaggccttgatgcatatttctaaagaatgggttttgaagcaataatgaatggcaaattctatttctccagtgacattagcattgtcaaaattgcccatctctgtacaggtgctgtcaatgctaattaaacttccgtgtctaaaacctccagagaatatggtactgggtgccggactggatgggagattctgttgcttcaaaatagggttagtagagcatttgggatcctcttgattgagaggtttcagaatatctggtgcactgaccttcctggtggtgacgttgaccgcagtgtcagactggctccgtctctctgtctgtcccacacactgcctggggcccgtggcgagaagatgcttctcagaagtcatatcattctgggatttggagagctcctgccaggactgcggctgcactggctctcgctgacaggaggtggagtaggaggaaccacagaaat

SEQ ID NO: 8906 - RNA, 2533 nt, Homo sapiens
  source 1..2533: mol_type = other RNA
acagggccgcagatggagactgctcaaggtcaaaggggtctccagctgggaccctgcacctggttcgtagcccctctgcagacgcacagtgcctcacgcctgctgcaacctggaaccttgaggccttcatgtcagtgcaggacaagagtcatgtctgtccatagattggggctggaaaggactttctgccactggagcttcgatagtgagcatgcatccccgccaacagctgtgtctccctttgaaccaagtctggttcctccaagcaagcggtcgttcattccaaagagggcctgatcccagacagttaactccaagcttgactgcctcagctgagctggggttacgccactgaagacaaatgagtgtttccactgggggcaagcctgcttcctcaggactggcgacttcagtctcagtttttgttggtctggcagagtgagacagcccttaacaaatgagttcaaggtgccatctggccgcacaggtaaattcttggctcctagcactaccaaacaaagttgaccatgaagtgatggctgatctgtcccttcttgagcctcttggagttttctgggccgtgaagggagaaccagcttagcccggactgtgagctctccattactctgaggaacgctgtcttcgtatttctccgccttggcccggagcggatgccagcggaaggactgtgttgtgctgtcttcaaagtcccacgtggccagaggaatgatcacttctccaagaaacactctccgggccagcgtgcccagatgccacaccgagacctgcagctgccgggtcaccagctgggcaggggccacctgatacttcaaggtctcctgaaaggtcgggtccacggtgttcctttggactccagtcttgcgctttccctgggaggatctgtcgggcaacaggtaggtcttcacatacggattgcactttttcttcttttcttctccataggcaaggttcttacaggccttgatgcatatttctaaagaatgggttttgaagcaataatgaatggcaaattctatttctccagtgacattagcattgtcaaaattgcccatctctgtacaggtgctgtcaatgctaattaaacttccgtgtctaaaacctccagagaatatggtactgggtgccggactggatgggagattctgttgcttcaaaatagggttagtagagcatttgggatcctcttgattgagaggtttcagaatatctggtgcactgaccttcctggtggtgacgttgaccgcagtgtcagactggctccgtctctctgtctgtcccacacactgcctggggcccgtggcgagaagatgcttctcagaagtcatatcattctgggatttggagagctttttcacgtgggtagcaagagacagaaacaaattttccacggacttattaaatcctctaaactgaccaaattcctgtaacctgccaggactgcggctgcactggctctcgctgacaggaggtggagtaggaggaaccacagaaattttgctcagcttctgataagattgcaagagctgccctccaactgtctcatgtttgcctccagttggaaatttcttggctcgttcctcatagaaccattctccagtttttattttgacattcctgtcctcgaagcacaccgtgcacttccaggcatgggtccccctcaggaacactcggcactgggcacacacgcggtggctgcagccccggcacacggcgccccggtgcagcaggaaccccagcacctgctggcagcgcgcacagcacttctctttgtgctcccagtccgtgttcttcgctcctttccaccggagatgctgcaggtgtgttttcagtttccgcccaaaggcaccgttttaaatgaataacaagagcggcctccctcctcctcctgagcgtcctctacgtttagttacataaggaggatcatctccaccaacagaccttcgttaggacccttctcaggcacgaagcccagcagcaggtgggtagtgatttgtaagcaaacagcattggcgacggagtggcaggccccaagcagagaaagctaaacacccaaagtgaccccccgggaagggcagcctaccgtgtcctctcctcctctgtgttttgaaccgcctggtctcggtacaggacctggagaatggcctcgcgttctaactccttgagagcactcagatctatttcttgggccatttcttctccgttttcgttgacccaggttggaagagcttcactgcatggaccaagcgctcacgccctgcagatgagcggcggaggccagctgcagccagccttgtttaaagagctccctctcctatttcactggcaactgttttgcttgtggttcttttttcctttttaactgtgtcatactccttagaagaagaaagcctcaagaagttctgcgtttgtcggagttacggctcgcagagcctcgtgctacccggggggtgttttcaccgggttctgcagcagctgctgacatccatctaagacaaaagcatatctcttttct

SEQ ID NO: 8907 - RNA, 2853 nt, Homo sapiens
  source 1..2853: mol_type = other RNA
acagggccgcagatggagactgctcaaggtcaaaggggtctccagctgggaccctgcacctggttcgtagcccctctgcagacgcacagtgcctcacgcctgctgcaacctggaaccttgaggccttcatgtcagtgcaggacaagagtcatgtctgtccatagattggggctggaaaggactttctgccactggagcttcgatagtgagcatgcatccccgccaacagctgtgtctccctttgaaccaagtctggttcctccaagcaagcggtcgttcattccaaagagggcctgatcccagacagttaactccaagcttgactgcctcagctgagctggggttacgccactgaagacaaatgagtgtttccactgggggcaagcctgcttcctcaggactggcgacttcagtctcagtttttgttggtctggcagagtgagacagcccttaacaaatgagttcaaggtgccatctggccgcacaggtaaattcttggctcctagcactaccaaacaaagttgaccatgaagtgatggctgatctgtcccttcttgagcctcttggagttttctgggccgtgaagggagaaccagcttagcccggactgtgagctctccattactctgaggaacgctgtcttcgtatttctccgccttggcccggagcggatgccagcggaaggactgtgttgtgctgtcttcaaagtcccacgtggccagaggaatgatcacttctccaagaaacactctccgggccagcgtgcccagatgccacaccgagacctgcagctgccgggtcaccagctgggcaggggccacctgatacttcaaggtctcctgaaaggtcgggtccacggtgttcctttggactccagtcttgcgctttccctgggaggatctgtcgggcaacaggtaggtcttcacatacggattgcactttttcttcttttcttctccataggcaaggttcttacaggccttgatgcatatttctaaagaatgggttttgaagcaataatgaatggcaaattctatttctccagtgacattagcattgtcaaaattgcccatctctgtacaggtgctgtcaatgctaattaaacttccgtgtctaaaacctccagagaatatggtactgggtgccggactggatgggagattctgttgcttcaaaatagggttagtagagcatttgggatcctcttgattgagaggtttcagaatatctggtgcactgaccttcctggtggtgacgttgaccgcagtgtcagactggctccgtctctctgtctgtcccacacactgcctggggcccgtggcgagaagatgcttctcagaagtcatatcattctgggatttggagagctttttcacgtgggtagcaagagacagaaacaaattttccacggacttattaaatcctctaaactgaccaaattcctgtaacctgccaggactgcggctgcactggctctcgctgacaggaggtggagtaggaggaaccacagaaattttgctcagcttctgataagattgcaagagctgccctccaactgtctcatgtttgcctccagttggaaatttcttggctcgttcctcatagaaccattctccagtttttattttgacattcctgtcctcgaagcacaccgtgcacttccaggcatgggtccccctcaggaacactcggcactgggcacacacgcggtggctgcagccccggcacacggcgccccggtgcagcaggaaccccagcacctgctggcagcgcgcacagcacttctctttgtgctcccagtccgtgttcttcgctcctttccaccggagatgctgcaggtgtgttttcagtttccgtgtcctctcctcctctgtgttttgaaccgcctggtctcggtacaggacctggagaatggcctcgcgttctaactccttgagagcactcagatctatttcttgggccatttcttctccgttttcgttgacccaggttggaagagcttcactgcatggaccaagcgctcacgccctgcagatgagcggcggaggccagctgcagccagccttgtttaaagagctccctctcctatttcactggcaactgttttgcttgtggttcttttttcctttttaactgtgtcatactccttagaagaagaaagcctcaagaagttctgcgtttgtcggagttacggctcgcagagcctcgtgctacccggggggtgttttcaccgggttctgcagcagctgctgacatccatctaagacaaaagcatatctcttttctgaggtttcaccagagattgttataaattatccacagctgcaagcagataatttctgcaaagcagaagtaattttcaagccaaggaaatttagaaatagcaataaaaagagtatcagtgactcatagaagctaaccttccatttaagatgtttccaggtcagcaggaaccatcatgaaaagctcagcccgttcaatacctggctgggctggtacctgactatgccagcaggggcaacgcctcttccctccttagatccaggttccagatgaacaggcagaactggcatccctcagtgccccaaggctctgagtctctgagagaggacaaagttgaacaggcgctttctctgaaagatcactgcaattcaccgctgattccgagtattctttctcattcggggagccgggcgcactgccttcagcagtcactttcgagtttgttgccaggtgtccgagcgggtttgaacgtccgcgtcaatccacacagtacaaaccggaggaggggccgggaccacgcttcccctccaggactgccttttgtacgtgtgttttgtttctgttgctaag

SEQ ID NO: 8908 - RNA, 2715 nt, Homo sapiens
  source 1..2715: mol_type = other RNA
acagggccgcagatggagactgctcaaggtcaaaggggtctccagctgggaccctgcacctggttcgtagcccctctgcagacgcacagtgcctcacgcctgctgcaacctggaaccttgaggccttcatgtcagtgcaggacaagagtcatgtctgtccatagattggggctggaaaggactttctgccactggagcttcgatagtgagcatgcatccccgccaacagctgtgtctccctttgaaccaagtctggttcctccaagcaagcggtcgttcattccaaagagggcctgatcccagacagttaactccaagcttgactgcctcagctgagctggggttacgccactgaagacaaatgagtgtttccactgggggcaagcctgcttcctcaggactggcgacttcagtctcagtttttgttggtctggcagagtgagacagcccttaacaaatgagttcaaggtgccatctggccgcacaggtaaattcttggctcctagcactaccaaacaaagttgaccatgaagtgatggctgatctgtcccttcttgagcctcttggagttttctgggccgtgaagggagaaccagcttagcccggactgtgagctctccattactctgaggaacgctgtcttcgtatttctccgccttggcccggagcggatgccagcggaaggactgtgttgtgctgtcttcaaagtcccacgtggccagaggaatgatcacttctccaagaaacactctccgggccagcgtgcccagatgccacaccgagacctgcagctgccgggtcaccagctgggcaggggccacctgatacttcaaggtctcctgaaaggtcgggtccacggtgttcctttggactccagtcttgcgctttccctgggaggatctgtcgggcaacaggtaggtcttcacatacggattgcactttttcttcttttcttctccataggcaaggttcttacaggccttgatgcatatttctaaagaatgggttttgaagcaataatgaatggcaaattctatttctccagtgacattagcattgtcaaaattgcccatctctgtacaggtgctgtcaatgctaattaaacttccgtgtctaaaacctccagagaatatggtactgggtgccggactggatgggagattctgttgcttcaaaatagggttagtagagcatttgggatcctcttgattgagaggtttcagaatatctggtgcactgaccttcctggtggtgacgttgaccgcagtgtcagactggctccgtctctctgtctgtcccacacactgcctggggcccgtggcgagaagatgcttctcagaagtcatatcattctgggatttggagagctttttcacgtgggtagcaagagacagaaacaaattttccacggacttattaaatcctctaaactgaccaaattcctgtaacctgccaggactgcggctgcactggctctcgctgacaggaggtggagtaggaggaaccacagaaattttgctcagcttctgataagattgcaagagctgccctccaactgtctcatgtttgcctccagttggaaatttcttggctcgttcctcatagaaccattctccagtttttattttgacattcctgtcctcgaagcacaccgtgcacttccaggcatgggtccccctcaggaacactcggcactgggcacacacgcggtggctgcagccccggcacacggcgccccggtgcagcaggaaccccagcacctgctggcagcgcgcacagcacttctctttgtgctcccagtccgtgttcttcgctcctttccaccggagatgctgcaggtgtgttttcagtttccgtgtcctctcctcctctgtgttttgaaccgcctggtctcggtacaggacctggagaatggcctcgcgttctaactccttgagagcactcagatctatttcttgggccatttcttctccgttttcgttgacccaggttggaagagcttcactgcatggaccaagcgctcacgccctgcagatgagcggcggaggccagctgcagccagccttgtttaaagagctccctctcctatttcactggcaactgttttgcttgtggttcttttttcctttttaactgtgtcatactccttagaagaagaaagcctcaagaagttctgcgtttgtcggagttacggctcgcagagcctcgtgctacccggggggtgttttcaccgggttctgcagcagctgctgacatccatctaagacaaaagcatatctcttttctgaggtttcaccagagattgttataaattatccacagctgcaagcagataatttctgcaaagcagaagtaattttcaagccaaggaaatttagaaatagcaataaaaagagtatcagtgactcatagaagctaaccttccatttaagatgtttccaggtcagcaggaaccatcatgaaaagctcagcccgttcaatacctggctgggctggtacctgactatgccagcaggggcaacgcctcttccctccttagatccaggttccagatgaacaggcagaactggcatccctcagtgccccaaggctctgagtctctgagagaggacaaagttgaacaggcgctttctctgaaagatcactgcaattcaccgctgattccgagtattctttctcattcggggagccttcgcatctgcttcaagagaagag

SEQ ID NO: 8909 - RNA, 2834 nt, Homo sapiens
  source 1..2834: mol_type = other RNA
acagggccgcagatggagactgctcaaggtcaaaggggtctccagctgggaccctgcacctggttcgtagcccctctgcagacgcacagtgcctcacgcctgctgcaacctggaaccttgaggccttcatgtcagtgcaggacaagagtcatgtctgtccatagattggggctggaaaggactttctgccactggagcttcgatagtgagcatgcatccccgccaacagctgtgtctccctttgaaccaagtctggttcctccaagcaagcggtcgttcattccaaagagggcctgatcccagacagttaactccaagcttgactgcctcagctgagctggggttacgccactgaagacaaatgagtgtttccactgggggcaagcctgcttcctcaggactggcgacttcagtctcagtttttgttggtctggcagagtgagacagcccttaacaaatgagttcaaggtgccatctggccgcacaggtaaattcttggctcctagcactaccaaacaaagttgaccatgaagtgatggctgatctgtcccttcttgagcctcttggagttttctgggccgtgaagggagaaccagcttagcccggactgtgagctctccattactctgaggaacgctgtcttcgtatttctccgccttggcccggagcggatgccagcggaaggactgtgttgtgctgtcttcaaagtcccacgtggccagaggaatgatcacttctccaagaaacactctccgggccagcgtgcccagatgccacaccgagacctgcagctgccgggtcaccagctgggcaggggccacctgatacttcaaggtctcctgaaaggtcgggtccacggtgttcctttggactccagtcttgcgctttccctgggaggatctgtcgggcaacaggtaggtcttcacatacggattgcactttttcttcttttcttctccataggcaaggttcttacaggccttgatgcatatttctaaagaatgggttttgaagcaataatgaatggcaaattctatttctccagtgacattagcattgtcaaaattgcccatctctgtacaggtgctgtcaatgctaattaaacttccgtgtctaaaacctccagagaatatggtactgggtgccggactggatgggagattctgttgcttcaaaatagggttagtagagcatttgggatcctcttgattgagaggtttcagaatatctggtgcactgaccttcctggtggtgacgttgaccgcagtgtcagactggctccgtctctctgtctgtcccacacactgcctggggcccgtggcgagaagatgcttctcagaagtcatatcattctgggatttggagagctttttcacgtgggtagcaagagacagaaacaaattttccacggacttattaaatcctctaaactgaccaaattcctgtaacctgccaggactgcggctgcactggctctcgctgacaggaggtggagtaggaggaaccacagaaattttgctcagcttctgataagattgcaagagctgccctccaactgtctcatgtttgcctccagttggaaatttcttggctcgttcctcatagaaccattctccagtttttattttgacattcctgtcctcgaagcacaccgtgcacttccaggcatgggtccccctcaggaacactcggcactgggcacacacgcggtggctgcagccccggcacacggcgccccggtgcagcaggaaccccagcacctgctggcagcgcgcacagcacttctctttgtgctcccagtccgtgttcttcgctcctttccaccggagatgctgcaggtgtgttttcagtttccgtgtcctctcctcctctgtgttttgaaccgcctggtctcggtacaggacctggagaatggcctcgcgttctaactccttgagagcactcagatctatttcttgggccatttcttctccgttttcgttgacccaggttggaagagcttcactgcatggaccaagcgctcacgccctgcagatgagcggcggaggccagctgcagccagccttgtttaaagagctccctctcctatttcactggcaactgttttgcttgtggttcttttttcctttttaactgtgtcatactccttagaagaagaaagcctcaagaagttctgcgtttgtcggagttacggctcgcagagcctcgtgctacccggggggtgttttcaccgggttctgcagcagctgctgacatccatctaagacaaaagcatatctcttttctgaggtttcaccagagattgttataaattatccacagctgcaagcagataatttctgcaaagcagaagtaattttcaagccaaggaaatttagaaatagcaataaaaagagtatcagtgactcatagaagctaaccttccatttaagatgtttccaggtcagcaggaaccatcatgaaaagctcagcccgttcaatacctggctgggctggtacctgactatgccagcaggggcaacgcctcttccctccttagatccaggttccagatgaacaggcagaactggcatccctcagtgccccaaggctctgagtctctggaaaacttaactccccaaagggaagtttcgttcagatagctaaagcatgccaatcccagtccccaagggaactgcaacaacgtctcaccgggcgcactgccttcagcagtcactttcgagtttgttgccaggtgtccgagcgggtttgaacgtccgcgtcaatccacacagtacaaaccggaggaggggccgggaccacgcttcccctccaggactgccttttgtacgtgt

SEQ ID NO: 8910 - RNA, 2945 nt, Homo sapiens
  source 1..2945: mol_type = other RNA
acagggccgcagatggagactgctcaaggtcaaaggggtctccagctgggaccctgcacctggttcgtagcccctctgcagacgcacagtgcctcacgcctgctgcaacctggaaccttgaggccttcatgtcagtgcaggacaagagtcatgtctgtccatagattggggctggaaaggactttctgccactggagcttcgatagtgagcatgcatccccgccaacagctgtgtctccctttgaaccaagtctggttcctccaagcaagcggtcgttcattccaaagagggcctgatcccagacagttaactccaagcttgactgcctcagctgagctggggttacgccactgaagacaaatgagtgtttccactgggggcaagcctgcttcctcaggactggcgacttcagtctcagtttttgttggtctggcagagtgagacagcccttaacaaatgagttcaaggtgccatctggccgcacaggtaaattcttggctcctagcactaccaaacaaagttgaccatgaagtgatggctgatctgtcccttcttgagcctcttggagttttctgggccgtgaagggagaaccagcttagcccggactgtgagctctccattactctgaggaacgctgtcttcgtatttctccgccttggcccggagcggatgccagcggaaggactgtgttgtgctgtcttcaaagtcccacgtggccagaggaatgatcacttctccaagaaacactctccgggccagcgtgcccagatgccacaccgagacctgcagctgccgggtcaccagctgggcaggggccacctgatacttcaaggtctcctgaaaggtcgggtccacggtgttcctttggactccagtcttgcgctttccctgggaggatctgtcgggcaacaggtaggtcttcacatacggattgcactttttcttcttttcttctccataggcaaggttcttacaggccttgatgcatatttctaaagaatgggttttgaagcaataatgaatggcaaattctatttctccagtgacattagcattgtcaaaattgcccatctctgtacaggtgctgtcaatgctaattaaacttccgtgtctaaaacctccagagaatatggtactgggtgccggactggatgggagattctgttgcttcaaaatagggttagtagagcatttgggatcctcttgattgagaggtttcagaatatctggtgcactgaccttcctggtggtgacgttgaccgcagtgtcagactggctccgtctctctgtctgtcccacacactgcctggggcccgtggcgagaagatgcttctcagaagtcatatcattctgggatttggagagctttttcacgtgggtagcaagagacagaaacaaattttccacggacttattaaatcctctaaactgaccaaattcctgtaacctgccaggactgcggctgcactggctctcgctgacaggaggtggagtaggaggaaccacagaaattttgctcagcttctgataagattgcaagagctgccctccaactgtctcatgtttgcctccagttggaaatttcttggctcgttcctcatagaaccattctccagtttttattttgacattcctgtcctcgaagcacaccgtgcacttccaggcatgggtccccctcaggaacactcggcactgggcacacacgcggtggctgcagccccggcacacggcgccccggtgcagcaggaaccccagcacctgctggcagcgcgcacagcacttctctttgtgctcccagtccgtgttcttcgctcctttccaccggagatgctgcaggtgtgttttcagtttccgtgtcctctcctcctctgtgttttgaaccgcctggtctcggtacaggacctggagaatggcctcgcgttctaactccttgagagcactcagatctatttcttgggccatttcttctccgttttcgttgacccaggttggaagagcttcactgcatggaccaagcgctcacgccctgcagatgagcggcggaggccagctgcagccagccttgtttaaagagctccctctcctatttcactggcaactgttttgcttgtggttcttttttcctttttaactgtgtcatactccttagaagaagaaagcctcaagaagttctgcgtttgtcggagttacggctcgcagagcctcgtgctacccggggggtgttttcaccgggttctgcagcagctgctgacatccatctaagacaaaagcatatctcttttctgaggtttcaccagagattgttataaattatccacagctgcaagcagataatttcttccatttaagatgtttccaggtcagcaggaaccatcatgaaaagctcagcccgttcaatacctggctgggctggtacctgactatgccagcaggggcaacgcctcttccctccttagatccaggttccagatgaacaggcagaactggcatccctcagtgccccaaggctctgagtctctgagagaggacaaagttgaacaggcgctttctctgaaagatcactgcaattcaccgctgattccgagtattctttctcattcggggagcctggaaaacttaactccccaaagggaagtttcgttcagatagctaaagcatgccaatcccagtccccaagggaactgcaacaacgtctcaccgggcgcactgccttcagcagtcactttcgagtttgttgccaggtgtccgagcgggtttgaacgtccgcgtcaatccacacagtacaaaccggaggaggggccgggaccacgcttcccctccaggactgccttttgtacgtgtgttttgtttctgttgctaaggtttagggagctgcccggctaccctcacggattcccatggaaactaccacctcccagaggacaggaggagaggcgaattcag

SEQ ID NO: 8911 - RNA, 2866 nt, Homo sapiens
  source 1..2866: mol_type = other RNA
acagggccgcagatggagactgctcaaggtcaaaggggtctccagctgggaccctgcacctggttcgtagcccctctgcagacgcacagtgcctcacgcctgctgcaacctggaaccttgaggccttcatgtcagtgcaggacaagagtcatgtctgtccatagattggggctggaaaggactttctgccactggagcttcgatagtgagcatgcatccccgccaacagctgtgtctccctttgaaccaagtctggttcctccaagcaagcggtcgttcattccaaagagggcctgatcccagacagttaactccaagcttgactgcctcagctgagctggggttacgccactgaagacaaatgagtgtttccactgggggcaagcctgcttcctcaggactggcgacttcagtctcagtttttgttggtctggcagagtgagacagcccttaacaaatgagttcaaggtgccatctggccgcacaggtaaattcttggctcctagcactaccaaacaaagttgaccatgaagtgatggctgatctgtcccttcttgagcctcttggagttttctgggccgtgaagggagaaccagcttagcccggactgtgagctctccattactctgaggaacgctgtcttcgtatttctccgccttggcccggagcggatgccagcggaaggactgtgttgtgctgtcttcaaagtcccacgtggccagaggaatgatcacttctccaagaaacactctccgggccagcgtgcccagatgccacaccgagacctgcagctgccgggtcaccagctgggcaggggccacctgatacttcaaggtctcctgaaaggtcgggtccacggtgttcctttggactccagtcttgcgctttccctgggaggatctgtcgggcaacaggtaggtcttcacatacggattgcactttttcttcttttcttctccataggcaaggttcttacaggccttgatgcatatttctaaagaatgggttttgaagcaataatgaatggcaaattctatttctccagtgacattagcattgtcaaaattgcccatctctgtacaggtgctgtcaatgctaattaaacttccgtgtctaaaacctccagagaatatggtactgggtgccggactggatgggagattctgttgcttcaaaatagggttagtagagcatttgggatcctcttgattgagaggtttcagaatatctggtgcactgaccttcctggtggtgacgttgaccgcagtgtcagactggctccgtctctctgtctgtcccacacactgcctggggcccgtggcgagaagatgcttctcagaagtcatatcattctgggatttggagagctttttcacgtgggtagcaagagacagaaacaaattttccacggacttattaaatcctctaaactgaccaaattcctgtaacctgccaggactgcggctgcactggctctcgctgacaggaggtggagtaggaggaaccacagaaattttgctcagcttctgataagattgcaagagctgccctccaactgtctcatgtttgcctccagttggaaatttcttggctcgttcctcatagaaccattctccagtttttattttgacattcctgtcctcgaagcacaccgtgcacttccaggcatgggtccccctcaggaacactcggcactgggcacacacgcggtggctgcagccccggcacacggcgccccggtgcagcaggaaccccagcacctgctggcagcgcgcacagcacttctctttgtgctcccagtccgtgttcttcgctcctttccaccggagatgctgcaggtgtgttttcagtttccgtgtcctctcctcctctgtgttttgaaccgcctggtctcggtacaggacctggagaatggcctcgcgttctaactccttgagagcactcagatctatttcttgggccatttcttctccgttttcgttgacccaggttggaagagcttcactgcatggaccaagcgctcacgccctgcagatgagcggcggaggccagctgcagccagccttgtttaaagagctccctctcctatttcactggcaactgttttgcttgtggttcttttttcctttttaactgtgtcatactccttagaagaagaaagcctcaagaagttctgcgtttgtcggagttacggctcgcagagcctcgtgctacccggggggtgttttcaccgggttctgcagcagctgctgacatccatcttccatttaagatgtttccaggtcagcaggaaccatcatgaaaagctcagcccgttcaatacctggctgggctggtacctgactatgccagcaggggcaacgcctcttccctccttagatccaggttccagatgaacaggcagaactggcatccctcagtgccccaaggctctgagtctctgagagaggacaaagttgaacaggcgctttctctgaaagatcactgcaattcaccgctgattccgagtattctttctcattcggggagcctggaaaacttaactccccaaagggaagtttcgttcagatagctaaagcatgccaatcccagtccccaagggaactgcaacaacgtctcaccgggcgcactgccttcagcagtcactttcgagtttgttgccaggtgtccgagcgggtttgaacgtccgcgtcaatccacacagtacaaaccggaggaggggccgggaccacgcttcccctccaggactgccttttgtacgtgtgttttgtttctgttgctaaggtttagggagctgcccggctaccctcacggattcccatggaaactaccacctcccagaggacaggaggagaggcgaattcag

SEQ ID NO: 8912 - RNA, 2634 nt, Homo sapiens
  source 1..2634: mol_type = other RNA
acagggccgcagatggagactgctcaaggtcaaaggggtctccagctgggaccctgcacctggttcgtagcccctctgcagacgcacagtgcctcacgcctgctgcaacctggaaccttgaggccttcatgtcagtgcaggacaagagtcatgtctgtccatagattggggctggaaaggactttctgccactggagcttcgatagtgagcatgcatccccgccaacagctgtgtctccctttgaaccaagtctggttcctccaagcaagcggtcgttcattccaaagagggcctgatcccagacagttaactccaagcttgactgcctcagctgagctggggttacgccactgaagacaaatgagtgtttccactgggggcaagcctgcttcctcaggactggcgacttcagtctcagtttttgttggtctggcagagtgagacagcccttaacaaatgagttcaaggtgccatctggccgcacaggtaaattcttggctcctagcactaccaaacaaagttgaccatgaagtgatggctgatctgtcccttcttgagcctcttggagttttctgggccgtgaagggagaaccagcttagcccggactgtgagctctccattactctgaggaacgctgtcttcgtatttctccgccttggcccggagcggatgccagcggaaggactgtgttgtgctgtcttcaaagtcccacgtggccagaggaatgatcacttctccaagaaacactctccgggccagcgtgcccagatgccacaccgagacctgcagctgccgggtcaccagctgggcaggggccacctgatacttcaaggtctcctgaaaggtcgggtccacggtgttcctttggactccagtcttgcgctttccctgggaggatctgtcgggcaacaggtaggtcttcacatacggattgcactttttcttcttttcttctccataggcaaggttcttacaggccttgatgcatatttctaaagaatgggttttgaagcaataatgaatggcaaattctatttctccagtgacattagcattgtcaaaattgcccatctctgtacaggtgctgtcaatgctaattaaacttccgtgtctaaaacctccagagaatatggtactgggtgccggactggatgggagattctgttgcttcaaaatagggttagtagagcatttgggatcctcttgattgagaggtttcagaatatctggtgcactgaccttcctggtggtgacgttgaccgcagtgtcagactggctccgtctctctgtctgtcccacacactgcctggggcccgtggcgagaagatgcttctcagaagtcatatcattctgggatttggagagctttttcacgtgggtagcaagagacagaaacaaattttccacggacttattaaatcctctaaactgaccaaattcctgtaacctgccaggactgcggctgcactggctctcgctgacaggaggtggagtaggaggaaccacagaaattttgctcagcttctgataagattgcaagagctgccctccaactgtctcatgtttgcctccagttggaaatttcttggctcgttcctcatagaaccattctccagtttttattttgacattcctgtcctcgaagcacaccgtgcacttccaggcatgggtccccctcaggaacactcggcactgggcacacacgcggtggctgcagccccggcacacggcgccccggtgcagcaggaaccccagcacctgctggcagcgcgcacagcacttctctttgtgctcccagtccgtgttcttcgctcctttccaccggagatgctgcaggtgtgttttcagtttccgtgtcctctcctcctctgtgttttgaaccgcctggtctcggtacaggacctggagaatggcctcgcgttctaactccttgagagcactcagatctatttcttgggccatttcttctccgttttcgttgacccaggttggaagagcttcactgcatggaccaagcgctcacgcccttccatttaagatgtttccaggtcagcaggaaccatcatgaaaagctcagcccgttcaatacctggctgggctggtacctgactatgccagcaggggcaacgcctcttccctccttagatccaggttccagatgaacaggcagaactggcatccctcagtgccccaaggctctgagtctctgagagaggacaaagttgaacaggcgctttctctgaaagatcactgcaattcaccgctgattccgagtattctttctcattcggggagcctggaaaacttaactccccaaagggaagtttcgttcagatagctaaagcatgccaatcccagtccccaagggaactgcaacaacgtctcaccgggcgcactgccttcagcagtcactttcgagtttgttgccaggtgtccgagcgggtttgaacgtccgcgtcaatccacacagtacaaaccggaggaggggccgggaccacgcttcccctccaggactgccttttgtacgtgtgttttgtttctgttgctaaggtttagggagctgcccggctaccctcacggattcccatggaaactaccacctcccagaggacaggaggagaggcgaattcag

SEQ ID NO: 8913 - RNA, 2323 nt, Homo sapiens
  source 1..2323: mol_type = other RNA
acagggccgcagatggagactgctcaaggtcaaaggggtctccagctgggaccctgcacctggttcgtagcccctctgcagacgcacagtgcctcacgcctgctgcaacctggaaccttgaggccttcatgtcagtgcaggacaagagtcatgtctgtccatagattggggctggaaaggactttctgccactggagcttcgatagtgagcatgcatccccgccaacagctgtgtctccctttgaaccaagtctggttcctccaagcaagcggtcgttcattccaaagagggcctgatcccagacagttaactccaagcttgactgcctcagctgagctggggttacgccactgaagacaaatgagtgtttccactgggggcaagcctgcttcctcaggactggcgacttcagtctcagtttttgttggtctggcagagtgagacagcccttaacaaatgagttcaaggtgccatctggccgcacaggtaaattcttggctcctagcactaccaaacaaagttgaccatgaagtgatggctgatctgtcccttcttgagcctcttggagttttctgggccgtgaagggagaaccagcttagcccggactgtgagctctccattactctgaggaacgctgtcttcgtatttctccgccttggcccggagcggatgccagcggaaggactgtgttgtgctgtcttcaaagtcccacgtggccagaggaatgatcacttctccaagaaacactctccgggccagcgtgcccagatgccacaccgagacctgcagctgccgggtcaccagctgggcaggggccacctgatacttcaaggtctcctgaaaggtcgggtccacggtgttcctttggactccagtcttgcgctttccctgggaggatctgtcgggcaacaggtaggtcttcacatacggattgcactttttcttcttttcttctccataggcaaggttcttacaggccttgatgcatatttctaaagaatgggttttgaagcaataatgaatggcaaattctatttctccagtgacattagcattgtcaaaattgcccatctctgtacaggtgctgtcaatgctaattaaacttccgtgtctaaaacctccagagaatatggtactgggtgccggactggatgggagattctgttgcttcaaaatagggttagtagagcatttgggatcctcttgattgagaggtttcagaatatctggtgcactgaccttcctggtggtgacgttgaccgcagtgtcagactggctccgtctctctgtctgtcccacacactgcctggggcccgtggcgagaagatgcttctcagaagtcatatcattctgggatttggagagctttttcacgtgggtagcaagagacagaaacaaattttccacggacttattaaatcctctaaactgaccaaattcctgtaacctgccaggactgcggctgcactggctctcgctgacaggaggtggagtaggaggaaccacagaaattttgctcagcttctgataagattgcaagagctgccctccaactgtctcatgtttgcctccagttggaaatttcttggctcgttcctcatagaaccattctccagtttttattttgacattcctgtcctcgaagcacaccgtgcacttccaggcatgggtccccctcaggaacactcggcactgggcacacacgcggtggctgcagccccggcacacggcgccccggtgcagcaggaaccccagcacctgctggcagcgcgcacagcacttctctttgtgctcccagtccgtgttcttcgctcctttccaccggagatgctgcaggtgtgttttcagtttccgtgtcctctcctcctctgtgttttgaaccgcctggtctcggtacaggacctggagaatggcctcgcgttctaactccttgagagcactcagatctatttcttgggccatttcttctccgttttcgttgacccaggttggaagagcttcactgcatggaccaagcgctcacgcccttccatttaagatgtttccaggtcagcaggaaccatcatgaaaagctcagcccgttcaatacctggctgggctggtacctgactatgccagcaggggcaacgcctcttccctccttagatccaggttccagatgaacaggcagaactggcatccctcagtgccccaaggctctgagtctctgagagaggacaaagttgaacaggcgctttctctgaaagatcactgcaattcaccgctgattccgagtattctttctcattcggggagccttcgcatctgcttcaagagaagag

SEQ ID NO: 8914 - RNA, 3034 nt, Homo sapiens
  source 1..3034: mol_type = other RNA
acagggccgcagatggagactgctcaaggtcaaaggggtctccagctgggaccctgcacctggttcgtagcccctctgcagacgcacagtgcctcacgcctgctgcaacctggaaccttgaggccttcatgtcagtgcaggacaagagtcatgtctgtccatagattggggctggaaaggactttctgccactggagcttcgatagtgagcatgcatccccgccaacagctgtgtctccctttgaaccaagtctggttcctccaagcaagcggtcgttcattccaaagagggcctgatcccagacagttaactccaagcttgactgcctcagctgagctggggttacgccactgaagacaaatgagtgtttccactgggggcaagcctgcttcctcaggactggcgacttcagtctcagtttttgttggtctggcagagtgagacagcccttaacaaatgagttcaaggtgccatctggccgcacaggtaaattcttggctcctagcactaccaaacaaagttgaccatgaagtgatggctgatctgtcccttcttgagcctcttggagttttctgggccgtgaagggagaaccagcttagcccggactgtgagctctccattactctgaggaacgctgtcttcgtatttctccgccttggcccggagcggatgccagcggaaggactgtgttgtgctgtcttcaaagtcccacgtggccagaggaatgatcacttctccaagaaacactctccgggccagcgtgcccagatgccacaccgagacctgcagctgccgggtcaccagctgggcaggggccacctgatacttcaaggtctcctgaaaggtcgggtccacggtgttcctttggactccagtcttgcgctttccctgggaggatctgtcgggcaacaggtaggtcttcacatacggattgcactttttcttcttttcttctccataggcaaggttcttacaggccttgatgcatatttctaaagaatgggttttgaagcaataatgaatggcaaattctatttctccagtgacattagcattgtcaaaattgcccatctctgtacaggtgctgtcaatgctaattaaacttccgtgtctaaaacctccagagaatatggtactgggtgccggactggatgggagattctgttgcttcaaaatagggttagtagagcatttgggatcctcttgattgagaggtttcagaatatctggtgcactgaccttcctggtggtgacgttgaccgcagtgtcagactggctccgtctctctgtctgtcccacacactgcctggggcccgtggcgagaagatgcttctcagaagtcatatcattctgggatttggagagctttttcacgtgggtagcaagagacagaaacaaattttccacggacttattaaatcctctaaactgaccaaattcctgtaacctgccaggactgcggctgcactggctctcgctgacaggaggtggagtaggaggaaccacagaaattttgctcagcttctgataagattgcaagagctgccctccaactgtctcatgtttgcctccagttggaaatttcttggctcgttcctcatagaaccattctccagtttttattttgacattcctgtcctcgaagcacaccgtgcacttccaggcatgggtccccctcaggaacactcggcactgggcacacacgcggtggctgcagccccggcacacggcgccccggtgcagcaggaaccccagcacctgctggcagcgcgcacagcacttctctttgtgctcccagtccgtgttcttcgctcctttccaccggagatgctgcaggtgtgttttcagtttcctgcagcccgtgtcctctcctcctctgtgttttgaaccgcctggtctcggtacaggacctggagaatggcctcgcgttctaactccttgagagcactcagatctatttcttgggccatttcttctccgttttcgttgacccaggttggaagagcttcactgcatggaccaagcgctcacgccctgcagatgagcggcggaggccagctgcagccagccttgtttaaagagctccctctcctatttcactggcaactgttttgcttgtggttcttttttcctttttaactgtgtcatactccttagaagaagaaagcctcaagaagttctgcgtttgtcggagttacggctcgcagagcctcgtgctacccggggggtgttttcaccgggttctgcagcagctgctgacatccatctaagacaaaagcatatctcttttctgaggtttcaccagagattgttataaattatccacagctgcaagcagataatttctgcaaagcagaagtaattttcaagccaaggaaatttagaaatagcaataaaaagagtatcagtgactcatagaagctaaccttccatttaagatgtttccaggtcagcaggaaccatcatgaaaagctcagcccgttcaatacctggctgggctggtacctgactatgccagcaggggcaacgcctcttccctccttagatccaggttccagatgaacaggcagaactggcatccctcagtgccccaaggctctgagtctctgagagaggacaaagttgaacaggcgctttctctgaaagatcactgcaattcaccgctgattccgagtattctttctcattcggggagcctggaaaacttaactccccaaagggaagtttcgttcagatagctaaagcatgccaatcccagtccccaagggaactgcaacaacgtctcaccgggcgcactgccttcagcagtcactttcgagtttgttgccaggtgtccgagcgggtttgaacgtccgcgtcaatccacacagtacaaaccggaggaggggccgggaccacgcttcccctccaggactgccttttgtacgtgtgttttgtttctgttgctaaggtttagggagctgcccggctaccctcacggattcccatggaaactaccacctcccagaggacaggaggagaggcgaattcag

SEQ ID NO: 8915 - RNA, 2371 nt, Homo sapiens
  source 1..2371: mol_type = other RNA
acagggccgcagatggagactgctcaaggtcaaaggggtctccagctgggaccctgcacctggttcgtagcccctctgcagacgcacagtgcctcacgcctgctgcaacctggaaccttgaggccttcatgtcagtgcaggacaagagtcatgtctgtccatagattggggctggaaaggactttctgccactggagcttcgatagtgagcatgcatccccgccaacagctgtgtctccctttgaaccaagtctggttcctccaagcaagcggtcgttcattccaaagagggcctgatcccagacagttaactccaagcttgactgcctcagctgagctggggttacgccactgaagacaaatgagtgtttccactgggggcaagcctgcttcctcaggactggcgacttcagtctcagtttttgttggtctggcagagtgagacagcccttaacaaatgagttcaaggtgccatctggccgcacaggtaaattcttggctcctagcactaccaaacaaagttgaccatgaagtgatggctgatctgtcccttcttgagcctcttggagttttctgggccgtgaagggagaaccagcttagcccggactgtgagctctccattactctgaggaacgctgtcttcgtatttctccgccttggcccggagcggatgccagcggaaggactgtgttgtgctgtcttcaaagtcccacgtggccagaggaatgatcacttctccaagaaacactctccgggccagcgtgcccagatgccacaccgagacctgcagctgccgggtcaccagctgggcaggggccacctgatacttcaaggtctcctgaaaggtcgggtccacggtgttcctttggactccagtcttgcgctttccctgggaggatctgtcgggcaacaggtaggtcttcacatacggattgcactttttcttcttttcttctccataggcaaggttcttacaggccttgatgcatatttctaaagaatgggttttgaagcaataatgaatggcaaattctatttctccagtgacattagcattgtcaaaattgcccatctctgtacaggtgctgtcaatgctaattaaacttccgtgtctaaaacctccagagaatatggtactgggtgccggactggatgggagattctgttgcttcaaaatagggttagtagagcatttgggatcctcttgattgagaggtttcagaatatctggtgcactgaccttcctggtggtgacgttgaccgcagtgtcagactggctccgtctctctgtctgtcccacacactgcctggggcccgtggcgagaagatgcttctcagaagtcatatcattctgggatttggagagctttttcacgtgggtagcaagagacagaaacaaattttccacggacttattaaatcctctaaactgaccaaattcctgtaacctgccaggactgcggctgcactggctctcgctgacaggaggtggagtaggaggaaccacagaaattttgctcagcttctgataagattgcaagagctgccctccaactgtctcatgtttgcctccagttggaaatttcttggctcgttcctcatagaaccattctccagtttttattttgacattcctgtcctcgaagcacaccgtgcacttccaggcatgggtccccctcaggaacactcggcactgggcacacacgcggtggctgcagccccggcacacggcgccccggtgcagcaggaaccccagcacctgctggcagcgcgcacagcacttctctttgtgctcccagtccgtgttcttcgctcctttccaccggagatgctgcaggtgtgttttcagtttcctgcagcccgtgtcctctcctcctctgtgttttgaaccgcctggtctcggtacaggacctggagaatggcctcgcgttctaactccttgagagcactcagatctatttcttgggccatttcttctccgttttcgttgacccaggttggaagagcttcactgcatggaccaagcgctcacgcccttccatttaagatgtttccaggtcagcaggaaccatcatgaaaagctcagcccgttcaatacctggctgggctggtacctgactatgccagcaggggcaacgcctcttccctccttagatccaggttccagatgaacaggcagaactggcatccctcagtgccccaaggctctgagtctctgagagaggacaaagttgaacaggcgctttctctgaaagatcactgcaattcaccgctgattccgagtattctttctcattcggggagccttcgcatctgcttcaagagaagagaccagagccggctctgcagagaaggaagtcaattcttctt

SEQ ID NO: 8916 - RNA, 2468 nt, Homo sapiens
  source 1..2468: mol_type = other RNA
acagggccgcagatggagactgctcaaggtcaaaggggtctccagctgggaccctgcacctggttcgtagcccctctgcagacgcacagtgcctcacgcctgctgcaacctggaaccttgaggccttcatgtcagtgcaggacaagagtcatgtctgtccatagattggggctggaaaggactttctgccactggagcttcgatagtgagcatgcatccccgccaacagctgtgtctccctttgaaccaagtctggttcctccaagcaagcggtcgttcattccaaagagggcctgatcccagacagttaactccaagcttgactgcctcagctgagctggggttacgccactgaagacaaatgagtgtttccactgggggcaagcctgcttcctcaggactggcgacttcagtctcagtttttgttggtctggcagagtgagacagcccttaacaaatgagttcaaggtgccatctggccgcacaggtaaattcttggctcctagcactaccaaacaaagttgaccatgaagtgatggctgatctgtcccttcttgagcctcttggagttttctgggccgtgaagggagaaccagcttagcccggactgtgagctctccattactctgaggaacgctgtcttcgtatttctccgccttggcccggagcggatgccagcggaaggactgtgttgtgctgtcttcaaagtcccacgtggccagaggaatgatcacttctccaagaaacactctccgggccagcgtgcccagatgccacaccgagacctgcagctgccgggtcaccagctgggcaggggccacctgatacttcaaggtctcctgaaaggtcgggtccacggtgttcctttggactccagtcttgcgctttccctgggaggatctgtcgggcaacaggtaggtcttcacatacggattgcactttttcttcttttcttctccataggcaaggttcttacaggccttgatgcatatttctaaagaatgggttttgaagcaataatgaatggcaaattctatttctccagtgacattagcattgtcaaaattgcccatctctgtacaggtgctgtcaatgctaattaaacttccgtgtctaaaacctccagagaatatggtactgggtgccggactggatgggagattctgttgcttcaaaatagggttagtagagcatttgggatcctcttgattgagaggtttcagaatatctggtgcactgaccttcctggtggtgacgttgaccgcagtgtcagactggctccgtctctctgtctgtcccacacactgcctggggcccgtggcgagaagatgcttctcagaagtcatatcattctgggatttggagagctttttcacgtgggtagcaagagacagaaacaaattttccacggacttattaaatcctctaaactgaccaaattcctgtaacctgccaggactgcggctgcactggctctcgctgacaggaggtggagtaggaggaaccacagaaattttgctcagcttctgataagattgcaagagctgccctccaactgtctcatgtttgcctccagttggaaatttcttggctcgttcctcatagaaccattctccagtttttattttgacattcctgtcctcgaagcacaccgtgcacttccaggcatgggtccccctcaggaacactcggcactgggcacacacgcggtggctgcagccccggcacacggcgccccggtgcagcaggaaccccagcacctgctggcagcgcgcacagcacttctctttgtgctcccagtccgtgttcttcgctcctttccaccggagatgctgcaggtgtgttttcagtttcctgcagcccttccatttaagatgtttccaggtcagcaggaaccatcatgaaaagctcagcccgttcaatacctggctgggctggtacctgactatgccagcaggggcaacgcctcttccctccttagatccaggttccagatgaacaggcagaactggcatccctcagtgccccaaggctctgagtctctgagagaggacaaagttgaacaggcgctttctctgaaagatcactgcaattcaccgctgattccgagtattctttctcattcggggagcctggaaaacttaactccccaaagggaagtttcgttcagatagctaaagcatgccaatcccagtccccaagggaactgcaacaacgtctcaccgggcgcactgccttcagcagtcactttcgagtttgttgccaggtgtccgagcgggtttgaacgtccgcgtcaatccacacagtacaaaccggaggaggggccgggaccacgcttcccctccaggactgccttttgtacgtgtgttttgtttctgttgctaaggtttagggagctgcccggctaccctcacggattcccatggaaactaccacctcccagaggacaggaggagaggcgaattcag

SEQ ID NO: 8917 - RNA, 2164 nt, Homo sapiens
  source 1..2164: mol_type = other RNA
acagggccgcagatggagactgctcaaggtcaaaggggtctccagctgggaccctgcacctggttcgtagcccctctgcagacgcacagtgcctcacgcctgctgcaacctggaaccttgaggccttcatgtcagtgcaggacaagagtcatgtctgtccatagattggggctggaaaggactttctgccactggagcttcgatagtgagcatgcatccccgccaacagctgtgtctccctttgaaccaagtctggttcctccaagcaagcggtcgttcattccaaagagggcctgatcccagacagttaactccaagcttgactgcctcagctgagctggggttacgccactgaagacaaatgagtgtttccactgggggcaagcctgcttcctcaggactggcgacttcagtctcagtttttgttggtctggcagagtgagacagcccttaacaaatgagttcaaggtgccatctggccgcacaggtaaattcttggctcctagcactaccaaacaaagttgaccatgaagtgatggctgatctgtcccttcttgagcctcttggagttttctgggccgtgaagggagaaccagcttagcccggactgtgagctctccattactctgaggaacgctgtcttcgtatttctccgccttggcccggagcggatgccagcggaaggactgtgttgtgctgtcttcaaagtcccacgtggccagaggaatgatcacttctccaagaaacactctccgggccagcgtgcccagatgccacaccgagacctgcagctgccgggtcaccagctgggcaggggccacctgatacttcaaggtctcctgaaaggtcgggtccacggtgttcctttggactccagtcttgcgctttccctgggaggatctgtcgggcaacaggtaggtcttcacatacggattgcactttttcttcttttcttctccataggcaaggttcttacaggccttgatgcatatttctaaagaatgggttttgaagcaataatgaatggcaaattctatttctccagtgacattagcattgtcaaaattgcccatctctgtacaggtgctgtcaatgctaattaaacttccgtgtctaaaacctccagagaatatggtactgggtgccggactggatgggagattctgttgcttcaaaatagggttagtagagcatttgggatcctcttgattgagaggtttcagaatatctggtgcactgaccttcctggtggtgacgttgaccgcagtgtcagactggctccgtctctctgtctgtcccacacactgcctggggcccgtggcgagaagatgcttctcagaagtcatatcattctgggatttggagagctttttcacgtgggtagcaagagacagaaacaaattttccacggacttattaaatcctctaaactgaccaaattcctgtaacctgccaggactgcggctgcactggctctcgctgacaggaggtggagtaggaggaaccacagaaattttgctcagcttctgataagattgcaagagctgccctccaactgtctcatgtttgcctccagttggaaatttcttggctcgttcctcatagaaccattctccagtttttattttgacattcctgtcctcgaagcacaccgtgcacttccaggcatgggtccccctcaggaacactcggcactgggcacacacgcggtggctgcagccccggcacacggcgccccggtgcagcaggaaccccagcacctgctggcagcgcgcacagcacttctctttgtgctcccagtccgtgttcttcgctcctttccaccggagatgctgcaggtgtgttttcagtttccttccatttaagatgtttccaggtcagcaggaaccatcatgaaaagctcagcccgttcaatacctggctgggctggtacctgactatgccagcaggggcaacgcctcttccctccttagatccaggttccagatgaacaggcagaactggcatccctcagtgccccaaggctctgagtctctgagagaggacaaagttgaacaggcgctttctctgaaagatcactgcaattcaccgctgattccgagtattctttctcattcggggagccttcgcatctgcttcaagagaagagaccagagccggctct

SEQ ID NO: 8918 - RNA, 1690 nt, Homo sapiens
  source 1..1690: mol_type = other RNA
acagggccgcagatggagactgctcaaggtcaaaggggtctccagctgggaccctgcacctggttcgtagcccctctgcagacgcacagtgcctcacgcctgctgcaacctggaaccttgaggccttcatgtcagtgcaggacaagagtcatgtctgtccatagattggggctggaaaggactttctgccactggagcttcgatagtgagcatgcatccccgccaacagctgtgtctccctttgaaccaagtctggttcctccaagcaagcggtcgttcattccaaagagggcctgatcccagacagttaactccaagcttgactgcctcagctgagctggggttacgccactgaagacaaatgagtgtttccactgggggcaagcctgcttcctcaggactggcgacttcagtctcagtttttgttggtctggcagagtgagacagcccttaacaaatgagttcaaggtgccatctggccgcacaggtaaattcttggctcctagcactaccaaacaaagttgaccatgaagtgatggctgatctgtcccttcttgagcctcttggagttttctgggccgtgaagggagaaccagcttagcccggactgtgagctctccattactctgaggaacgctgtcttcgtatttctccgccttggcccggagcggatgccagcggaaggactgtgttgtgctgtcttcaaagtcccacgtggccagaggaatgatcacttctccaagaaacactctccgggccagcgtgcccagatgccacaccgagacctgcagctgccgggtcaccagctgggcaggggccacctgatacttcaaggtctcctgaaaggtcgggtccacggtgttcctttggactccagtcttgcgctttccctgggaggatctgtcgggcaacaggtaggtcttcacatacggattgcactttttcttcttttcttctccataggcaaggttcttacaggccttgatgcatatttctaaagaatgggttttgaagcaataatgaatggcaaattctatttctccagtgacattagcattgtcaaaattgcccatctctgtacaggtgctgtcaatgctaattaaacttccgtgtctaaaacctccagagaatatggtactgggtgccggactggatgggagattctgttgcttcaaaatagggttagtagagcatttgggatcctcttgattgagaggtttcagaatatctggtgcactgaccttctctggggcgtggacagggtgtggttggtctctggagcaggcttcacctagctcttggtcatctctttgccccagtgtccctgtctttagtagggacaggaacagtaccaacttcatagggctgtcttaaggattacaaaggctaaatacctctgaagggcattacgctgagaacaatgccaggcatctggttaaccccaagtcagtgttagcctctgagtggtttcctgtgactcaagcaagtaagataattactcatgcttccacacgccccttcctgaaccctctttcttcagcggtcctcatttgtccttcttatgggaacatagagtttagaattcagagtcaaatcccaggtctgctcctggctccatctctcattcactatgtgacattaggcacgttggtcaacctctcactaaaactcaggcttttttttttttttt

SEQ ID NO: 8919 - RNA, 151 nt, Homo sapiens
  source 1..151: mol_type = other RNA
acaggtgaggttcttgggagcctggcgtctggcccaaccacacacctggggaattgctggcctgacttctgacccctgactcctcatacccttcctccagagcatgacatttgaccaccaactgaaacctgacctctgaccccagaccact

SEQ ID NO: 8920 - RNA, 1644 nt, Homo sapiens
  source 1..1644: mol_type = other RNA
acagtctgctgaggttggagcacagggaatgggaggaggcacaggccttgaggcaggtgccaccctgggcccgctgcagctgaacctccagcagagccttggtgccctccaggctggtgagcgttgtcagcagctcatcccgctccgcctccaggccccgcacctgcttgcggtactggtccttctcgatgaggctctgtgagtactgcaactggatccggtcacggctctggatggcctggtctcgctccttctcaatctcctccagttgggccaggacagtggccatgcggtgcttgtacaggtcacagtccttctgcagcgtgcggtgcttgagccgcaggtcttccatctcctgcaggtactggtcgcgcagctcctcggcccactgcagctccccctgcacggcatgcagcttctggcacagctcctgcctgctgtcctgcgcctcccgccagtcatgctctaggatgtccagcaggatgcgctcggagcccggggcccccggccggctcgcctcctgctgcaggccctcctgcaactcccgcagtgacgccgtcagccgctggttctcagcacgcagctcagagacaaggtccacattgtctggctccttctccttctccttctccttctccttctcctctgccccagggggcgggcccctggcccttcgaagcagtgcacactcttcctccagccgactcactttgagcttgagctgatccaccgccagctgcaggtcacggctgcgaagtacagccgagttcttctcctcactgagctgtgccaggcgcatggcgatcatgtagttctcatccttgagccgcagcagctccaggctgcccgcctcccagtcctcccgcagccgttgacagcgctcctgagcctgctgctggtcccgcagccgctgctccagccctgcccgctcctcctcgagcacccggccccgggcctgcagttgctgctcccgctgcagctggctcttgcgagcttcccgcagccgtcgcacctctgtcatcaagaattgggtcaggccctcaggcccctcctcatcgaggatcatggagcagcgctgggcgggttcctggcccgtgagcagcgtgaagtgttcggggtagtagaactccagggcttccaggaaggcctcatagcccctcttgccacggcagcgcaagatgtccatcaggcgcccggtgcggttgacgcggcacgggaagcggtaggtgctcagcacctcctcctcgtcctgctcgtcgatgacccggcactggcgcagatacggcgtgagcttggccgggttcagggcgcgagccagccgatgccggacgccctcgattcgctcccacagcgcgtcctcctccgcctcagaccccgagccggccccggcctcctcctcggcctcccccgcctccgcccggcccggcatggccgtgtcctcagggtctgcgggcaagaggcgcacgggggtcgaccagggctccctagggctagatgtgcggccaagcacccccggggcgtcgtccgcagacccgccgtcgggggcgcgccccgagctccccgcgactcaccccgcacgctacagtcgcctcgggctcccgggtccgcactcgggcggcggctccgccggcgcaggggggcggt

SEQ ID NO: 8921 - RNA, 3575 nt, Homo sapiens
  source 1..3575: mol_type = other RNA
acagtctgctgaggttggagctgagggtggaaggggagtgagctgacgctcggaaggtgtcttgagattatcatccgctgagggtggaagcggcccccgcagacgctcggcaggtgtcttgatattatcatctgctgagggtggagctgagggtggaaggggagtgagctgacgctcggaaggtgtcttgagattatcatcggctgagggtggaagcggcccccgcagacgctcggcaggtgtcttgatattatcatctgctgagggtggagctgagggtggaaggggagtgagctgacgtttggaaggtgtcttgagattatcatcggctgagggtggaagcggcccccgcagacgccacagacgctccccgcagacgctcggcaggtgtcttgatattatcatctgctgagggtggagctgagggtggaaggggagtgagctgacgctcggaaggtgtcttgagattatcatcggctgagggtggaagcggcccccgcagacgctcggcaggtgtcttgatattatcatctgctgagggtggagctgagggtggaaggggagtgagctgacgctcggaaggtgtcttgagattatcatcggctgagggtggaagcggcccccgcagacgctcggcaggtgtcttgatattatcatctgctgagggtggagctgagggtggaaggggagtgagctgacgctcggaaggtgtcttgagattatcatcggctgagggtggaagcggcccccgcagacgctcggcaggtgtcttgatattatcatctgctgagggtggagctgagggtggaaggggagtgagctgacgctcggaaggtgtcttgagattatcatcggctgagggtggaagcggcccccgcagacgctcggcaggtgtcttgatattatcatctgctgagggtggagctgagggtggaaggggagtgagctgacgctcggaaggtgtcttgagattatcatcggctgagggtggaagcggcccccgcagacgctcggcaggtgtcttgatattatcatctgctgagggtggagctgagggtggaaggggagtgagctgacgctcggaaggtgtcttgagattatcatccgctgacggtggaagcggaacccgcagatgctcagcaggtatcttgatattatcatctgctgagggtggagctgagggtggaaggggagtgagctgacgctcggaaggtctcttgagattatcatccgctgagggtggaagcggaactgcagatgctcggcaggtgtcttgatattatcatctgctgagggtggagctgagggtggaaggggagtgagctgacgctcggaaggtgtcttgagattatcatccgctgagggtggaagcggcccccgcagatgctcggcagttgtcttgatattatcatctgctgagggtggagctgagggtggaaggggagtgagctgacgctcagaaggtgtcttgagattatcatccgctgagggtggaagcggcccccgcagatgctcggcaggtgtcttgatattatcatctgctgagggtggagctgagggtggaaggggagtgagctgacgctcagaaggtgtcttgagattatcatcggctgagggtggaagcggcccccgcagacgctcggcaggtgtcttgatattatcatctgctgagggtggagctgagggtggaaggggagtgagctgacgctcagaaggtgtcttgagattatcatccgctgagggtggaagcggcccccgcagatgctcggcaggtgtcttgatattatcatctgctgagggtggagctgagggtggaaggggagtgagctgacgctcagaaggtgtcttgagattatcatccgctgagggtggaagcggcccccgcagacgctcggcagttgtcttgatattatcatctgctgagggtggagctgagggtggaaggggagtgagctgacgctcggaaggtgtcttgagattatcatccgctgagggtggaaggggatggagcagacactcggcacgtgtcttgagattatcatccgctgagggtggagctgagggtggagctgagggtggaaggggagtgagcagacactcgggaggtgtcttgagattatcatccgctgagggtggaaggggagtgagcagacactcgggaggtgtcttgagattatcatccgctgagggtggaaggggagtgagcagacactcgagaggtgtcttgaggctcagggagttatcagttatacaatgttgttgagttggaggaggtggctggtggcccatcctgttttttaaagtttcagctgtgaggtagggccagtagggcaatcctgaagaatgacgatgctccgctgccgccattctgacccagttgcaaagagcctttcttgcagaaggggggattttgcatttgtggtagtcctctgcccgccgccgcaactcttgcgcacgttgaaacattttctgttttctggcggtcttcctctttccattgattttgtcatgacggttgattttcgttgtcaccttcctcttacggattttagctctaacttttgtttccacatgcctccgtagagtaatgacgtctttcaggccaattttatttcctcgaaaggaagaaactcttttctttgtgtgcatacaaatggacctcagcccttcctgtctacggcggttggacctccaggctctctgctgtacatccgtggatccatcatgtccatttcgagaccagaagatagtcttcaggagagacacccaaaggtaaactatccagagggtaatgacaactttataacttgtcggaaacgcaataataatatgtaaccaaggacttccaccaaagtcagtcccacgatgatgatggtcagccagagtattgataacctgatttctggtcctccccaaccagctccctgtccctgcttctgggcgctccttccttcctgagctcccagggttcctcaaggtcaccttcctcaggtactcgcatgggcatgtcactgactttacgtgctgctgcagctccttggtgagctggccctggtcatgggacaggaactgtggggtcaggacaatagagagcttcaccatttgcagaatgagaacaggggctcatgatgagtgccaacctcagttttcttctgtgtgaaacaggaacaatagtttcattcgtcattcagtttctctcaaggtttcacgagatcatacctataaaacatccaagtcatttaaatgtatcatcatttctgtcataattagtgggatccatttcactattattggatatacagttctgtgcctgaaacctacaaaaaaagaaaatgttaagtctaaaaagcattagtgatttctcatttttatattactaattataaccctatttaatcacacaaggccttgtccgtggcaggtgctcaataaacacttgtcgaatcaatgcatgtgggctccggagccacactgtttagattctattctgcctccaccacttatcagctgtgtgatctgggtaagataattcacctctttatgtctgcacttccctctccataaactatatataa

SEQ ID NO: 8922 - RNA, 3713 nt, Homo sapiens
  source 1..3713: mol_type = other RNA
acagtctgctgaggttggagctgagggtggaaggggagtgagctgacgctcggaaggtgtcttgagattatcatccgctgagggtggaagcggcccccgcagacgctcggcaggtgtcttgatattatcatctgctgagggtggagctgagggtggaaggggagtgagctgacgctcggaaggtgtcttgagattatcatcggctgagggtggaagcggcccccgcagacgctcggcaggtgtcttgatattatcatctgctgagggtggagctgagggtggaaggggagtgagctgacgtttggaaggtgtcttgagattatcatcggctgagggtggaagcggcccccgcagacgctcggcaggtgtcttgatattatcatctgctgagggtggagctgagggtggaaggggagtgagctgacgtttggaaggtgtcttgagattatcatccgctgagggtggaagcggaacccacagacgctccccgcagacgctcggcaggtgtcttgatattatcatctgctgagggtggagctgagggtggaaggggagtgagctgacgctcggaaggtgtcttgagattatcatcggctgagggtggaagcggcccccgcagacgctcggcaggtgtcttgatattatcatctgctgagggtggagctgagggtggaaggggagtgagctgacgctcggaaggtgtcttgagattatcatcggctgagggtggaagcggcccccgcagacgctcggcaggtgtcttgatattatcatctgctgagggtggagctgagggtggaaggggagtgagctgacgctcggaaggtgtcttgagattatcatcggctgagggtggaagcggcccccgcagacgctcggcaggtgtcttgatattatcatctgctgagggtggagctgagggtggaaggggagtgagctgacgctcggaaggtgtcttgagattatcatcggctgagggtggaagcggcccccgcagacgctcggcaggtgtcttgatattatcatctgctgagggtggagctgagggtggaaggggagtgagctgacgctcggaaggtgtcttgagattatcatcggctgagggtggaagcggcccccgcagacgctcggcaggtgtcttgatattatcatctgctgagggtggagctgagggtggaaggggagtgagctgacgctcggaaggtgtcttgagattatcatccgctgacggtggaagcggaacccgcagatgctcagcaggtatcttgatattatcatctgctgagggtggagctgagggtggaaggggagtgagctgacgctcggaaggtctcttgagattatcatccgctgagggtggaagcggaactgcagatgctcggcaggtgtcttgatattatcatctgctgagggtggagctgagggtggaaggggagtgagctgacgctcggaaggtgtcttgagattatcatccgctgagggtggaagcggcccccgcagatgctcggcagttgtcttgatattatcatctgctgagggtggagctgagggtggaaggggagtgagctgacgctcagaaggtgtcttgagattatcatccgctgagggtggaagcggcccccgcagatgctcggcaggtgtcttgatattatcatctgctgagggtggagctgagggtggaaggggagtgagctgacgctcagaaggtgtcttgagattatcatcggctgagggtggaagcggcccccgcagacgctcggcaggtgtcttgatattatcatctgctgagggtggagctgagggtggaaggggagtgagctgacgctcagaaggtgtcttgagattatcatccgctgagggtggaagcggcccccgcagatgctcggcaggtgtcttgatattatcatctgctgagggtggagctgagggtggaaggggagtgagctgacgctcagaaggtgtcttgagattatcatccgctgagggtggaagcggcccccgcagacgctcggcagttgtcttgatattatcatctgctgagggtggagctgagggtggaaggggagtgagctgacgctcggaaggtgtcttgagattatcatccgctgagggtggaaggggatggagcagacactcggcacgtgtcttgagattatcatccgctgagggtggagctgagggtggagctgagggtggaaggggagtgagcagacactcgggaggtgtcttgagattatcatccgctgagggtggaaggggagtgagcagacactcgggaggtgtcttgagattatcatccgctgagggtggaaggggagtgagcagacactcgagaggtgtcttgaggctcagggagttatcagttatacaatgttgttgagttggaggaggtggctggtggcccatcctgttttttaaagtttcagctgtgaggtagggccagtagggcaatcctgaagaatgacgatgctccgctgccgccattctgacccagttgcaaagagcctttcttgcagaaggggggattttgcatttgtggtagtcctctgcccgccgccgcaactcttgcgcacgttgaaacattttctgttttctggcggtcttcctctttccattgattttgtcatgacggttgattttcgttgtcaccttcctcttacggattttagctctaacttttgtttccacatgcctccgtagagtaatgacgtctttcaggccaattttatttcctcgaaaggaagaaactcttttctttgtgtgcatacaaatggacctcagcccttcctgtctacggcggttggacctccaggctctctgctgtacatccgtggatccatcatgtccatttcgagaccagaagatagtcttcaggagagacacccaaaggtaaactatccagagggtaatgacaactttataacttgtcggaaacgcaataataatatgtaaccaaggacttccaccaaagtcagtcccacgatgatgatggtcagccagagtattgataaccttcctcaggtactcgcatgggcatgtcactgactttacgtgctgctgcagctccttggtgagctggccctggtcatgggacaggaactgtggggtcaggacaatagagagcttcaccatttgcagaatgagaacaggggctcatgatgagtgccaacctcagttttcttctgtgtgaaacaggaacaatagtttcattcgtcattcagtttctctcaaggtttcacgagatcatacctataaaacatccaagtcatttaaatgtatcatcatttctgtcataattagtgggatccatttcactattattggatatacagttctgtgcctgaaacctacaaaaaaagaaaatgttaagtctaaaaagcattagtgatttctcatttttatattactaattataaccctatttaatcacacaaggccttgtccgtggcaggtgctcaataaacacttgtcgaatcaatgcatgtgggctccggagccacactgtttagattctattctgcctccaccacttatcagctgtgtgatctgggtaagataattcacctctttatgtctgcacttccctctccataaactatatataatgagaatccttagctcattcggttgtggtgaggggtgaatgatttggcacacaggaggggcttgttaaacattagctgtgatgatctccttccaaatcttcattttca

SEQ ID NO: 8923 - RNA, 47 nt, Homo sapiens
  source 1..47: mol_type = other RNA
acatcgccccaccttccccagatgcctgccttgctcagccccacgta

SEQ ID NO: 8924 - RNA, 224 nt, Homo sapiens
  source 1..224: mol_type = other RNA
acatcgccccaccttccccagcgcagtcttcgccccttgcataggaggccacatctcctacacgtagatatgcagagagcgtgtcaacgcgcaagagctgcagcgccccatttaaccaccaagaggctccagggccgctggttaaaatcgtgcgggaagagatagcttgacgccaggagttcaagaccggcccgagcaaaatagtgacccacccccaacccccg

SEQ ID NO: 8925 - RNA, 560 nt, Homo sapiens
  source 1..560: mol_type = other RNA
acatcgccccaccttccccaggcacacaggtacaagcacttcagtgggctgctgggtacgtgcaaaagtggtaagtggtcagcaaaagaatgctgtcctgagtttttccacatcagtgatttttcttgctgtgagttctttaccaatccagatggggcatcatcacttgtgacttgtatatggaagtcagtgggacttcatagtggaagtgacatttgtgccaggtcttttggcaaatctgggtgactttgactggaacacctaatattctggtccagcgactctaccggtgggtggtgtatcttcgcctgtagactgggagtttcttgaggtcaggggagtgacttgcctatctttgcctcttagccttagcagatccccagtagacagctgacactcagaaccgaccaaaagaaggaaggaatgggacctcctgaggaagggcacagaactgtcctgtaaatggaaactagaccggacgcacgccaagccgatgacccacagtaacaggtgttctccatctctgatgtctgtgattcatcctgcacagctgcgcgcac

SEQ ID NO: 8926 - RNA, 861 nt, Homo sapiens
  source 1..861: mol_type = other RNA
acatcgccccaccttccccagggctgctcttggggacgcagcaggacaggcggctcccctttctaaggggagataggtgctgtcaccaacgaggaagggaagtgaagaggataccctcccaagaggctctcctgggcacagccaaagcccagccaggccaccaagatctgagacgcttccacttgtccaggctgaggcagccatgggacccctcccctcttcgtgcccctaaacacacgctgatgtctgccttcaggtgctgagcggggtcctggtaaaacggctaatctccaaatacgaaagattgcctgcacatccatttttcttgttttctgagacagggtctccctctgtcgcccaggctggagtgcagtggtgcgaatacagctcactgcagcctccacctcctgggctccagccatcctcctgcttcagcctctcgagtagctatgaccacagccactcgctaccacggccatacggggtctatgttgcccaggctggtctggaactcctggcttcaagcgatcctctcacctcagcctctcttaagtgctgggattacaggcatgagcccccttgtccatccgcacaccacacccacttctgaagagcacctgggtagactggccccctcccacaactctggccctctccgtggctgcagggagctttgccgaagtggggatgtgagccacccttgggatgggggacagagaccccaccccactcccctgccctgtccccacccccatgaggaccaccaccaaaggtctagttgaaagagagtgacatcggtggggcgcggtggctcacacctgtaatcccagcactttgaaaagttcgaggcgggcggatcgc

SEQ ID NO: 8927 - RNA, 1242 nt, Homo sapiens
  source 1..1242: mol_type = other RNA
acatcgccccaccttccccagggctgctcttggggacgcagcaggacaggcggctcccctttctaaggggagataggtgctgtcaccaacgaggaagggaagtgaagaggataccctcccaagaggctctcctgggcacagccaaagcccagccaggccaccaagatctgagacgcttccacttgtccaggctgaggcagccatgggacccctcccctcttcgtgcccctaaacacacgctgatgtctgccttcaggtgctgagcggggtcctggtaaaacggctaatctccaaatacgaaagattgcctgcacatccatttttcttgttttctgagacagggtctccctctgtcgcccaggctggagtgcagtggtgcgaatacagctcactgcagcctccacctcctgggctccagccatcctcctgcttcagcctctcgagtagctatgaccacagccactcgctaccacggccatacggggtctatgttgcccaggctggtctggaactcctggcttcaagcgatcctctcacctcagcctctcttaagtgctgggattacaggcatgagcccccttgtccatccgcacaccacacccacttctgaagagcacctgggtagactggccccctcccacaactctggccctctccgtggctgcagggagctttgccgaagtggggatgtgagccacccttgggatgggggacagagaccccaccccactcccctgccctgtccccacccccatgaggaccaccaccaaaggtctagttgaaagagagtgacatcggtggggcgcggtggctcacacctgtaatcccagcactttgaaaagttcgaggcgggcggatcgcctgaggtcaggagttcgagaccagcctggccaacatggggaaacgctgtctctactaaaaatacaacaattagccaggcgtggtggtgcgtgcctgtagtcccagctactcaggaggctgaggcaggagaatcacttgaaccggggaggcggaggttgcggtgagtggagattgcgccactgcactccagcctgcgtggcagagcaagactccatctcaaaaaaaataaagagggtgaaacagggatagaagcatgacagacccgtcacctccctgcccatacataccaggtggcccgctgggtaaggtggtgatccctgggagcagggccagcagcagcacggtgcccagcatgctggaccagctgaggtcggagtgttt

SEQ ID NO: 8928 - RNA, 140 nt, Homo sapiens
  source 1..140: mol_type = other RNA
acatcgccccaccttccccagtgagggtcccgcgcggcacgccgcccctgccagtccggccgcctagctccagcgccgggccgcgccgacctgcctggcccgccgtcccgccgcggcggcccctcctccgccgtccgggc

SEQ ID NO: 8929 - RNA, 37 nt, Homo sapiens
  source 1..37: mol_type = other RNA
accaggaggctgaggcccctgcctgttgctcggtggt

SEQ ID NO: 8930 - RNA, 1436 nt, Homo sapiens
  source 1..1436: mol_type = other RNA
accaggaggctgaggcccctgcctgttgctcggtggtctgcagttctgtcccgggctcagagctgcctccttttgactcaggcaacaggagctcctgggcagcatcttcagtcctagaatggccttcaccagcagaggtggggggaccggtcccctcctgggacaggcctctgcccccagaggggatggaagcgtcctggtcctccccttccgtgtggtcctggaattgcgggctgctctgagcctcacttcctgtggccactcctgcctctcccaaagcctgggcctgcagggggctgtcgccaacctcggtgggcgcggagaggccgtcaccctccagtggcgtggtggctgtgcctgggggctggctcggctggccagtggggccactctgctgggcttggctgtggggcagggctgtgtcctgaggccacgggtttgaaagcaaagtcaggtgacaggggctggcaggagaaaggggcaaggaagccagctctgaggaagcggacttgttccccttctttttcttcttccttttcttctttttgctctgctcacagtctgcagaaggcacgctggcggcctcaagcggggctgcatcctgcttccttctcttgctgggtatggcattagcagcttcccattcatcggatatgaggtctacagcagcatctaccaaaacctctgatgtagctccttcttggacggtccaggaggctttggaacagggctcctcggggttttcttgccaactgtctgagcccgggaacaagcacgggcccccttcctccttcagctcctgcccacactccatttcaccctccgaggccgacgccattgtggagttattgttctcagaatctgctatgggggctgcaggaggcagcctctctccgcactggctgcagaacttgggggtttcctccttggagacatgctggcacgaaggacactccatgggtcctgctgggactgccctgcagatccagaagcaagagcaggagtcgctggcagcctgctatatactacatgtcctgtcacgtgaccacggcttcagtttcattttcctggccttgagccccgcgctcgggcgacttcgccaagtcggaaggacgctgcgcggtgcggttcagacggggcgatgcctccctcgtaaaagttaggagtctgtttttgcaacttcacttttccgttgttgccattcgtacaggcgcaggattcccgggcggacctgcaggcccgggtccggctgtccccttccactacaccccccgtgccccggccacttcccgggggcagcactgccggggcgcaaagcctcctccgcgctctgcgctccggggatgtcgccggggtcccaggcgtgcccgctgcccccaccccgacccctcccgcagccggggaacagggtcagtgggcgccgcgggcggggctgg

SEQ ID NO: 8931 - RNA, 1149 nt, Homo sapiens
  source 1..1149: mol_type = other RNA
accaggaggctgaggcccctgcctgttgctcggtggtctgcagttctgtcccgggctcagagctgcctccttttgactcaggcaacaggagctcctgggcagcatcttcagtcctagaatggccttcaccagcagaggtggggggaccggtcccctcctgggacaggcctctgcccccagaggggatggaagcgtcctggtcctccccttccgtgtggtcctggaattgcgggctgctctgagcctcacttcctgtggccactcctgcctctcccaaagcctgggcctgcagggggctgtcgccaacctcggtgggcgcggagaggccgtcaccctccagtggcgtggtggctgtgcctgggggctggctcggctggccagtggggccactctgctgggcttggctgtggggcagggctgtgtcctgaggccacgggtttgaaagcaaagtcaggtgacaggggctggcaggagaaaggggcaaggaagccagctctgaggaagcggacttgttccccttctttttcttcttccttttcttctttttgctctgctcacagtctgcagaaggcacgctggcggcctcaagcggggctgcatcctgcttccttctcttgctgggtatggcattagcagcttcccattcatcggatatgaggtctacagcagcatctaccaaaacctctgatgtagctccttcttggacggtccaggaggctttggaacagggctcctcggggttttcttgccaactgtctgagcccgggaacaagcacgggcccccttcctccttcagctcctgcccacactccatttcaccctccgaggccgacgccattgtggagttattgttctcagaatctgctatgggggctgcaggaggcagcctctctccgcactggctgcagaacttgggggtttcctccttggagacatgctggcacgaaggacactccatgggtcctgctgggactgccctgcagatccagaagcaagagcaggagtcgctggcagcctgctatatactacatgtcctgtcacgtgaccacggcttcagtttcattttctgcggcccccgagctcgccgcctgccgcgcgctgtcgcccctcgggtcacggggccctgggccccgccctgcccgccgccgc

SEQ ID NO: 8932 - RNA, 1053 nt, Homo sapiens
  source 1..1053: mol_type = other RNA
accaggaggctgaggcccctgcctgttgctcggtggtctgcagttctgtcccgggctcagagctgcctccttttgactcaggcaacaggagctcctgggcagcatcttcagtcctagaatggccttcaccagcagaggtggggggaccggtcccctcctgggacaggcctctgcccccagaggggatggaagcgtcctggtcctccccttccgtgtggtcctggaattgcgggctgctctgagcctcacttcctgtggccactcctgcctctcccaaagcctgggcctgcagggggctgtcgccaacctcggtgggcgcggagaggccgtcaccctccagtggcgtggtggctgtgcctgggggctggctcggctggccagtggggccactctgctgggcttggctgtggggcagggctgtgtcctgaggccacgggtttgaaagcaaagtcaggtgacaggggctggcaggagaaaggggcaaggaagccagctctgaggaagcggacttgttccccttctttttcttcttccttttcttctttttgctctgctcacagtctgcagaaggcacgctggcggcctcaagcggggctgcatcctgcttccttctcttgctgggtatggcattagcagcttcccattcatcggatatgaggtctacagcagcatctaccaaaacctctgatgtagctccttcttggacggtccaggaggctttggaacagggctcctcggggttttcttgccaactgtctgagcccgggaacaagcacgggcccccttcctccttcagctcctgcccacactccatttcaccctccgaggccgacgccattgtggagttattgttctcagaatctgctatgggggctgcaggaggcagcctctctccgcactggctgcagaacttgggggtttcctccttggagacatgctggcacgaaggacactccatgggtcctgctgggactgccctgcggcccccgagctcgccgcctgccgcgcgctgtcgcccctcgggtcacggggccctgggccccgccctgcccg

SEQ ID NO: 8933 - RNA, 970 nt, Homo sapiens
  source 1..970: mol_type = other RNA
accaggaggctgaggcccctgcctgttgctcggtggtctgcagttctgtcccgggctcagagctgcctccttttgactcaggcaacaggagctcctgggcagcatcttcagtcctagaatggccttcaccagcagaggtggggggaccggtcccctcctgggacaggcctctgcccccagaggggatggaagcgtcctggtcctccccttccgtgtggtcctggaattgcgggctgctctgagcctcacttcctgtggccactcctgcctctcccaaagcctgggcctgcagggggctgtcgccaacctcggtgggcgcggagaggccgtcaccctccagtggcgtggtggctgtgcctgggggctggctcggctggccagtggggccactctgctgggcttggctgtggggcagggctgtgtcctgaggccacgggtttgaaagcaaagtcaggtgacaggggctggcaggagaaaggggcaaggaagccagctctgaggaagcggacttgttccccttctttttcttcttccttttcttctttttgctttcttggacggtccaggaggctttggaacagggctcctcggggttttcttgccaactgtctgagcccgggaacaagcacgggcccccttcctccttcagctcctgcccacactccatttcaccctccgaggccgacgccattgtggagttattgttctcagaatctgctatgggggctgcaggaggcagcctctctccgcactggctgcagaacttgggggtttcctccttggagacatgctggcacgaaggacactccatgggtcctgctgggactgccctgcagatccagaagcaagagcaggagtcgctggcagcctgctatatactacatgtcctgtcacgtgaccacggcttcagtttcattttctgcggcccccgagctcgccgcctgccgcgcgctgtcgcccctcgggtcac

SEQ ID NO: 8934 - RNA, 2551 nt, Homo sapiens
  source 1..2551: mol_type = other RNA
accaggaggctgaggccccttgggggtatcattctgtttctggaaggcagctttctcaaaaggctgctctggcaactgctgcttctcaacccccttggcccttccaaggggctgatgatggtccttaggtttcagggtggcctgagtcttggatggggataacacagccggtgtttgtgtgtctgtgcccttgggaggggcattctgcctgaggaaagcaactttcttggaggactgtaatttaggtgatcgttgctttagcttcccagtcacctttggctccctgatcccttcggcttttccagctggctgactgctatcctggaagctggaggaagcttgggtctttgtgacagaaggtacagtggacaattctgagtctgcccctttggagatgccattcagcttctggaaggaggccttcttgggatgttgctgtttctgcagctgctgctttgtctttgcagcccccttggctttcttggctggctggctgctgttctcagacttggggatgacctgaggcaagtctacatttgtaggtgtggctgtttcagaatttcctgtaatcctagctacttgggagtctgaggcacaagaatcgcttgaacctggaaggtggaggttgcaatgagctgagattgcaccactgcagtccagcctgagcgacaaagcaagacaccgtctgtctgggactgagggatagaattggaaaatttcttgaacttggcaatgaagaacccatccatattgtgggtatgagggtagaagcgtcgggtagaacgcagactggggtggaagcgcctttctcgaaagcgggtaaaaccttcctggccaaagtctaggcccgtgggcaccagtcgcacattcctctttttcagagcatagtctaccacccactcattctcttctactgtgatagaacaggtgcagtaaaccaggtagcctcctgtcttggaggtcgcattgacagagtcaatagcactcaggagcaactccttctggaggtgagcacagcgcaggatgtccttctcatccttgttagtcttcacggctggatccttggagatgaccccagtgccactgcagggagcatccagcagtactcggtcaaagccccccaccaccttggggaactggcgcccatcatagtggctgataatggtgttggtgactcccagccgatgcaagttgcccacaacactcttgagccgctcagcattggcgtcattggcaaggatcacacccgtgttcttcatcagctgggccatgtagctggtctttcctccaggggcacaacacatgtccaggatccgctcatgttcctggggtgccaaggccatgacgggcaacatgctggaggctccctgcagcatgtagtgcccagccaggtactcgggggtagcaccaatgggcacagaagaatcatacaccactagtccagtctttgaccacttgcccaggggatccaggttaaccccacgattgattagagcctgtgcaaggtctcggcgtcgggttttcaaggtattggtccggagggtgacgggccgaggcacctcattagcttctaagaactccaccagctcagacagagggaagaggtccatgagcttgccaagcaggaagtctccataggagtagtaaatggccagatccttcttgagccggttcaggtattcagaacgagaccgcccttcctcccgctgagccccaaaatcacgcagaattcccacaatatcctggatccgcttgtgaactcgttgcaggtctggagcctgggcatcctgctccatctccccagcagggggcagcacaaatggttcctcatccacattgatctgcaggcccccatctgcctcttccacctttggggggcctgactcaggggtcacttctttctcttcctcctcgtcctcggtctcctcttcactccactggatcccagcagcagcttcccgggccttctgcttccgagcagctctttcaatgggcagcaacgcttcaccttcctcctcatcctcagagttggagtcagctccatagtcatctaccgtatcagcatcgtcctcggagccccagaggtccccgtggttcaccataccatcttcttcagagtcttcctcctcctcttcctcatcactgccaggtgctgggcgcttcttgcctcgaggagcattaaatagggactggggtcccttcttaccagctgtctggacagctccttttggtagctttccaggcaatggtttggcctcaggagacttatttgtcttaggggcttcaacagagcccaatctcctcttggctgccctctttcgagcacgactagacagcctcttggaattttcgtcacttactgcaggcaagaatctgacgagttctgtctcggcacccttctgcttccgggcctttcggcctggcccccgcttctccttcgtagggtccaacttgcgccccatggtacagaatgcgggttaatgtccgagagtgcccttcgggcggccctccacgtgcaatccggacctagctttcggccggcactcgccac

SEQ ID NO: 8935 - RNA, 2441 nt, Homo sapiens
  source 1..2441: mol_type = other RNA
accaggaggctgaggccccttgggggtatcattctgtttctggaaggcagctttctcaaaaggctgctctggcaactgctgcttctcaacccccttggcccttccaaggggctgatgatggtccttaggtttcagggtggcctgagtcttggatggggataacacagccggtgtttgtgtgtctgtgcccttgggaggggcattctgcctgaggaaagcaactttcttggaggactgtaatttaggtgatcgttgctttagcttcccagtcacctttggctccctgatcccttcggcttttccagctggctgactgctatcctggaagctggaggaagcttgggtctttgtgacagaaggtacagtggacaattctgagtctgcccctttggagatgccattcagcttctggaaggaggccttcttgggatgttgctgtttctgcagctgctgctttgtctttgcagcccccttggctttcttggctggctggctgctgttctcagacttggggatgacctgaggcaagtctacatttgtaggtgtggctgtttcagaatttcctgtctgggactgagggatagaattggaaaatttcttgaacttggcaatgaagaacccatccatattgtgggtatgagggtagaagcgtcgggtagaacgcagactggggtggaagcgcctttctcgaaagcgggtaaaaccttcctggccaaagtctaggcccgtgggcaccagtcgcacattcctctttttcagagcatagtctaccacccactcattctcttctactgtgatagaacaggtgcagtaaaccaggtagcctcctgtcttggaggtcgcattgacagagtcaatagcactcaggagcaactccttctggaggtgagcacagcgcaggatgtccttctcatccttgttagtcttcacggctggatccttggagatgaccccagtgccactgcagggagcatccagcagtactcggtcaaagccccccaccaccttggggaactggcgcccatcatagtggctgataatggtgttggtgactcccagccgatgcaagttgcccacaacactcttgagccgctcagcattggcgtcattggcaaggatcacacccgtgttcttcatcagctgggccatgtagctggtctttcctccaggggcacaacacatgtccaggatccgctcatgttcctggggtgccaaggccatgacgggcaacatgctggaggctccctgcagcatgtagtgcccagccaggtactcgggggtagcaccaatgggcacagaagaatcatacaccactagtccagtctttgaccacttgcccaggggatccaggttaaccccacgattgattagagcctgtgcaaggtctcggcgtcgggttttcaaggtattggtccggagggtgacgggccgaggcacctcattagcttctaagaactccaccagctcagacagagggaagaggtccatgagcttgccaagcaggaagtctccataggagtagtaaatggccagatccttcttgagccggttcaggtattcagaacgagaccgcccttcctcccgctgagccccaaaatcacgcagaattcccacaatatcctggatccgcttgtgaactcgttgcaggtctggagcctgggcatcctgctccatctccccagcagggggcagcacaaatggttcctcatccacattgatctgcaggcccccatctgcctcttccacctttggggggcctgactcaggggtcacttctttctcttcctcctcgtcctcggtctcctcttcactccactggatcccagcagcagcttcccgggccttctgcttccgagcagctctttcaatgggcagcaacgcttcaccttcctcctcatcctcagagttggagtcagctccatagtcatctaccgtatcagcatcgtcctcggagccccagaggtccccgtggttcaccataccatcttcttcagagtcttcctcctcctcttcctcatcactgccaggtgctgggcgcttcttgcctcgaggagcattaaatagggactggggtcccttcttaccagctgtctggacagctcctgcagagatcccttttggtagctttccaggcaatggtttggcctcaggagacttatttgtcttaggggcttcaacagagcccaatctcctcttggctgccctctttcgagcacgactagacagcctcttggaattttcgtcacttactgcaggcaagaatctgacgagttctgtctcggcacccttctgcttccgggcctttcggcctggcccccgcttctccttcgtagggtccaacttgcgccccatggtacagaatgcgggttaatgtccgagagtgcccttcgggcggccctccacgtgcaatccggacctagctttcggccggcactcgccac

SEQ ID NO: 8936 - RNA, 2509 nt, Homo sapiens
  source 1..2509: mol_type = other RNA
accaggaggctgaggccccttgggggtatcattctgtttctggaaggcagctttctcaaaaggctgctctggcaactgctgcttctcaacccccttggcccttccaaggggctgatgatggtccttaggtttcagggtggcctgagtcttggatggggataacacagccggtgtttgtgtgtctgtgcccttgggaggggcattctgcctgaggaaagcaactttcttggaggactgtaatttaggtgatcgttgctttagcttcccagtcacctttggctccctgatcccttcggcttttccagctggctgactgctatcctggaagctggaggaagcttgggtctttgtgacagaaggtacagtggacaattctgagtctgcccctttggagatgccattcagcttctggaaggaggccttcttgggatgttgctgtttctgcagctgctgctttgtctttgcagcccccttggctttcttggctggctggctgctgttctcagacttggggatgacctgaggcaagtctacatttgtaggtgtggctgtttcagaatttcctgtctgggactgagggatagaattggaaaatttcttgaacttggcaatgaagaacccatccatattgtgggtatgagggtagaagcgtcgggtagaacgcagactggggtggaagcgcctttctcgaaagcgggtaaaaccttcctggccaaagtctaggcccgtgggcaccagtcgcacattcctctttttcagagcatagtctaccacccactcattctcttctactgtgatagaacaggtgcagtaaaccaggtagcctcctgtcttggaggtcgcattgacagagtcaatagcactcaggagcaactccttctggaggtgagcacagcgcaggatgtccttctcatccttgttagtcttcacggctggatccttggagatgaccccagtgccactgcagggagcatccagcagtactcggtcaaagccccccaccaccttggggaactggcgcccatcatagtggctgataatggtgttggtgactcccagccgatgcaagttgcccacaacactcttgagccgctcagcattggcgtcattggcaaggatcacacccgtgttcttcatcagctgggccatgtagctggtctttcctccaggggcacaacacatgtccaggatccgctcatgttcctggggtgccaaggccatgacgggcaacatgctggaggctccctgcagcatgtagtgcccagccaggtactcgggggtagcaccaatgggcacagaagaatcatacaccactagtccagtctttgaccacttgcccaggggatccaggttaaccccacgattgattagagcctgtgcaaggtctcggcgtcgggttttcaaggtattggtccggagggtgacgggccgaggcacctcattagcttctaagaactccaccagctcagacagagggaagaggtccatgagcttgccaagcaggaagtctccataggagtagtaaatggccagatccttcttgagccggttcaggtattcagaacgagaccgcccttcctcccgctgagccccaaaatcacgcagaattcccacaatatcctggatccgcttgtgaactcgttgcaggtctggagcctgggcatcctgctccatctccccagcagggggcagcacaaatggttcctcatccacattgatctgcaggcccccatctgcctcttccacctttggggggcctgactcaggggtcacttctttctcttcctcctcgtcctcggtctcctcttcactccactggatcccagcagcagcttcccgggccttctgcttccgagcagctctttcaatgggcagcaacgcttcaccttcctcctcatcctcagagttggagtcagctccatagtcatctaccgtatcagcatcgtcctcggagccccagaggtccccgtggttcaccataccatcttcttcagagtcttcctcctcctcttcctcatcactgccaggtgctgggcgcttcttgcctcgaggagcattaaatagggactggggtcccttcttaccagctgtctggacagctcctgcagagatcccttttggtagctttccaggcaatggtttggcctcaggagacttatttgtcttaggggcttcaacagagcccaatctcctcttggctgccctctttcgagcacgactagacagcctcttggaattttcgtcacttactgcaggcaagaatctgacgagttctgtctcggcacccttctgcttccgggcctttcggcctggcccccgcttctccttcgtagggtccaacttgcgccccatggtaccttctccccacgtcccagaccaggtcagtgctgccactcttcgtcccccaatttcctctagacccaccagaatgcgggttaatgtccgagagtgcccttcgggcggccctccacgtgcaatccggacctagctttcggccggcactcgccac

SEQ ID NO: 8937 - RNA, 2429 nt, Homo sapiens
  source 1..2429: mol_type = other RNA
accaggaggctgaggccccttgggggtatcattctgtttctggaaggcagctttctcaaaaggctgctctggcaactgctgcttctcaacccccttggcccttccaaggggctgatgatggtccttaggtttcagggtggcctgagtcttggatggggataacacagccggtgtttgtgtgtctgtgcccttgggaggggcattctgcctgaggaaagcaactttcttggaggactgtaatttaggtgatcgttgctttagcttcccagtcacctttggctccctgatcccttcggcttttccagctggctgactgctatcctggaagctggaggaagcttgggtctttgtgacagaaggtacagtggacaattctgagtctgcccctttggagatgccattcagcttctggaaggaggccttcttgggatgttgctgtttctgcagctgctgctttgtctttgcagcccccttggctttcttggctggctggctgctgttctcagacttggggatgacctgaggcaagtctacatttgtaggtgtggctgtttcagaatttcctgtctgggactgagggatagaattggaaaatttcttgaacttggcaatgaagaacccatccatattgtgggtatgagggtagaagcgtcgggtagaacgcagactggggtggaagcgcctttctcgaaagcgggtaaaaccttcctggccaaagtctaggcccgtgggcaccagtcgcacattcctctttttcagagcatagtctaccacccactcattctcttctactgtgatagaacaggtgcagtaaaccaggtagcctcctgtcttggaggtcgcattgacagagtcaatagcactcaggagcaactccttctggaggtgagcacagcgcaggatgtccttctcatccttgttagtcttcacggctggatccttggagatgaccccagtgccactgcagggagcatccagcagtactcggtcaaagccccccaccaccttggggaactggcgcccatcatagtggctgataatggtgttggtgactcccagccgatgcaagttgcccacaacactcttgagccgctcagcattggcgtcattggcaaggatcacacccgtgttcttcatcagctgggccatgtagctggtctttcctccaggggcacaacacatgtccaggatccgctcatgttcctggggtgccaaggccatgacgggcaacatgctggaggctccctgcagcatgtagtgcccagccaggtactcgggggtagcaccaatgggcacagaagaatcatacaccactagtccagtctttgaccacttgcccaggggatccaggttaaccccacgattgattagagcctgtgcaaggtctcggcgtcgggttttcaaggtattggtccggagggtgacgggccgaggcacctcattagcttctaagaactccaccagctcagacagagggaagaggtccatgagcttgccaagcaggaagtctccataggagtagtaaatggccagatccttcttgagccggttcaggtattcagaacgagaccgcccttcctcccgctgagccccaaaatcacgcagaattcccacaatatcctggatccgcttgtgaactcgttgcaggtctggagcctgggcatcctgctccatctccccagcagggggcagcacaaatggttcctcatccacattgatctgcaggcccccatctgcctcttccacctttggggggcctgactcaggggtcacttctttctcttcctcctcgtcctcggtctcctcttcactccactggatcccagcagcagcttcccgggccttctgcttccgagcagctctttcaatgggcagcaacgcttcaccttcctcctcatcctcagagttggagtcagctccatagtcatctaccgtatcagcatcgtcctcggagccccagaggtccccgtggttcaccataccatcttcttcagagtcttcctcctcctcttcctcatcactgccaggtgctgggcgcttcttgcctcgaggagcattaaatagggactggggtcccttcttaccagctgtctggacagctccttttggtagctttccaggcaatggtttggcctcaggagacttatttgtcttaggggcttcaacagagcccaatctcctcttggctgccctctttcgagcacgactagacagcctcttggaattttcgtcacttactgcaggcaagaatctgacgagttctgtctcggcacccttctgcttccgggcctttcggcctggcccccgcttctccttcgtagggtccaacttgcgccccatggtacagaatgcgggttaatgtccgagagtgcccttcgggcggccctccacgtgcaatccggacctagctttcggccggcactcgccac

SEQ ID NO: 8938 - RNA, 2497 nt, Homo sapiens
  source 1..2497: mol_type = other RNA
accaggaggctgaggccccttgggggtatcattctgtttctggaaggcagctttctcaaaaggctgctctggcaactgctgcttctcaacccccttggcccttccaaggggctgatgatggtccttaggtttcagggtggcctgagtcttggatggggataacacagccggtgtttgtgtgtctgtgcccttgggaggggcattctgcctgaggaaagcaactttcttggaggactgtaatttaggtgatcgttgctttagcttcccagtcacctttggctccctgatcccttcggcttttccagctggctgactgctatcctggaagctggaggaagcttgggtctttgtgacagaaggtacagtggacaattctgagtctgcccctttggagatgccattcagcttctggaaggaggccttcttgggatgttgctgtttctgcagctgctgctttgtctttgcagcccccttggctttcttggctggctggctgctgttctcagacttggggatgacctgaggcaagtctacatttgtaggtgtggctgtttcagaatttcctgtctgggactgagggatagaattggaaaatttcttgaacttggcaatgaagaacccatccatattgtgggtatgagggtagaagcgtcgggtagaacgcagactggggtggaagcgcctttctcgaaagcgggtaaaaccttcctggccaaagtctaggcccgtgggcaccagtcgcacattcctctttttcagagcatagtctaccacccactcattctcttctactgtgatagaacaggtgcagtaaaccaggtagcctcctgtcttggaggtcgcattgacagagtcaatagcactcaggagcaactccttctggaggtgagcacagcgcaggatgtccttctcatccttgttagtcttcacggctggatccttggagatgaccccagtgccactgcagggagcatccagcagtactcggtcaaagccccccaccaccttggggaactggcgcccatcatagtggctgataatggtgttggtgactcccagccgatgcaagttgcccacaacactcttgagccgctcagcattggcgtcattggcaaggatcacacccgtgttcttcatcagctgggccatgtagctggtctttcctccaggggcacaacacatgtccaggatccgctcatgttcctggggtgccaaggccatgacgggcaacatgctggaggctccctgcagcatgtagtgcccagccaggtactcgggggtagcaccaatgggcacagaagaatcatacaccactagtccagtctttgaccacttgcccaggggatccaggttaaccccacgattgattagagcctgtgcaaggtctcggcgtcgggttttcaaggtattggtccggagggtgacgggccgaggcacctcattagcttctaagaactccaccagctcagacagagggaagaggtccatgagcttgccaagcaggaagtctccataggagtagtaaatggccagatccttcttgagccggttcaggtattcagaacgagaccgcccttcctcccgctgagccccaaaatcacgcagaattcccacaatatcctggatccgcttgtgaactcgttgcaggtctggagcctgggcatcctgctccatctccccagcagggggcagcacaaatggttcctcatccacattgatctgcaggcccccatctgcctcttccacctttggggggcctgactcaggggtcacttctttctcttcctcctcgtcctcggtctcctcttcactccactggatcccagcagcagcttcccgggccttctgcttccgagcagctctttcaatgggcagcaacgcttcaccttcctcctcatcctcagagttggagtcagctccatagtcatctaccgtatcagcatcgtcctcggagccccagaggtccccgtggttcaccataccatcttcttcagagtcttcctcctcctcttcctcatcactgccaggtgctgggcgcttcttgcctcgaggagcattaaatagggactggggtcccttcttaccagctgtctggacagctccttttggtagctttccaggcaatggtttggcctcaggagacttatttgtcttaggggcttcaacagagcccaatctcctcttggctgccctctttcgagcacgactagacagcctcttggaattttcgtcacttactgcaggcaagaatctgacgagttctgtctcggcacccttctgcttccgggcctttcggcctggcccccgcttctccttcgtagggtccaacttgcgccccatggtaccttctccccacgtcccagaccaggtcagtgctgccactcttcgtcccccaatttcctctagacccaccagaatgcgggttaatgtccgagagtgcccttcgggcggccctccacgtgcaatccggacctagctttcggccggcactcgccac

SEQ ID NO: 8939 - RNA, 2540 nt, Homo sapiens
  source 1..2540: mol_type = other RNA
accaggaggctgaggccccttgggggtatcattctgtttctggaaggcagctttctcaaaaggctgctctggcaactgctgcttctcaacccccttggcccttccaaggggctgatgatggtccttaggtttcagggtggcctgagtcttggatggggataacacagccggtgtttgtgtgtctgtgcccttgggaggggcattctgcctgaggaaagcaactttcttggaggactgtaatttaggtgatcgttgctttagcttcccagtcacctttggctccctgatcccttcggcttttccagctggctgactgctatcctggaagctggaggaagcttgggtctttgtgacagaaggtacagtggacaattctgagtctgcccctttggagatgccattcagcttctggaaggaggccttcttgggatgttgctgtttctgcagctgctgctttgtctttgcagcccccttggctttcttggctggctggctgctgttctcagacttggggatgacctgaggcaagtctacatttgtaggtgtggctgtttcagaatttcctgtctgggactgagggatagaattggaaaatttcttgaacttggcaatgaagaacccatccatattgtgggtatgagggtagaagcgtcgggtagaacgcagactggggtggaagcgcctttctcgaaagcgggtaaaaccttcctggccaaagtctaggcccgtgggcaccagtcgcacattcctctttttcagagcatagtctaccacccactcattctcttctactgtgatagaacaggtgcagtaaaccaggtagcctcctgtcttggaggtcgcattgacagagtcaatagcactcaggagcaactccttctggaggtgagcacagcgcaggatgtccttctcatccttgttagtcttcacggctggatccttggagatgaccccagtgccactgcagggagcatccagcagtactcggtcaaagccccccaccaccttggggaactggcgcccatcatagtggctgataatggtgttggtgactcccagccgatgcaagttgcccacaacactcttgagccgctcagcattggcgtcattggcaaggatcacacccgtgttcttcatcagctgggccatgtagctggtctttcctccaggggcacaacacatgtccaggatccgctcatgttcctggggtgccaaggccatgacgggcaacatgctggaggctccctgcagcatgtagtgcccagccaggtactcgggggtagcaccaatgggcacagaagaatcatacaccactagtccagtctttgaccacttgcccaggggatccaggttaaccccacgattgattagagcctgtgcaaggtctcggcgtcgggttttcaaggtattggtccggagggtgacgggccgaggcacctcattagcttctaagaactccaccagctcagacagagggaagaggtccatgagcttgccaagcaggaagtctccataggagtagtaaatggccagatccttcttgagccggttcaggtattcagaacgagaccgcccttcctcccgctgagccccaaaatcacgcagaattcccacaatatcctggatccgcttgtgaactcgttgcaggtctggagcctgggcatcctgctccatctccccagcagggggcagcacaaatggttcctcatccacattgatctgcaggcccccatctgcctcttccacctttggggggcctgactcaggggtcacttctttctcttcctcctcgtcctcggtctcctcttcactccactggatcccagcagcagcttcccgggccttctgcttccgagcagctctttcaatgggcagcaactgtaaatcccagctacttgggaagctgaggcaggagaattgcttgaacccgggaggtggaggttgcagtgagccaagaccgagccactgcactccagccgcttcaccttcctcctcatcctcagagttggagtcagctccatagtcatctaccgtatcagcatcgtcctcggagccccagaggtccccgtggttcaccataccatcttcttcagagtcttcctcctcctcttcctcatcactgccaggtgctgggcgcttcttgcctcgaggagcattaaatagggactggggtcccttcttaccagctgtctggacagctcctgcagagatcccttttggtagctttccaggcaatggtttggcctcaggagacttatttgtcttaggggcttcaacagagcccaatctcctcttggctgccctctttcgagcacgactagacagcctcttggaattttcgtcacttactgcaggcaagaatctgacgagttctgtctcggcacccttctgcttccgggcctttcggcctggcccccgcttctccttcgtagggtccaacttgcgccccatggtacagaatgcgggttaatgtccgagagtgcccttcgggcggccctccacgtgcaatccggacctagctttcggccggcactcgccac

SEQ ID NO: 8940 - RNA, 322 nt, Homo sapiens
  source 1..322: mol_type = other RNA
accccactcctggtaccaaaatctgtattagtcagggttcttttttgctgaaggaggttcttgccttgatgttgatggctgctgactgatcaagatggcggctgctgaaggttggaatggctgtagcaatttctttacaatgttgctgtggactgtccttgtgtacagacagtcctgaggttctgaacttcagtcctttacgttaagacttctcctttttctcctttcctgatgaggaaatggctccctccaaatcccatcctctcacaaacctttgggtttcctgtagtcccagctactcgggaggctgaggcaggagaat

SEQ ID NO: 8941 - RNA, 2406 nt, Homo sapiens
  source 1..2406: mol_type = other RNA
accccactcctggtaccctcccacccaggctcaacccgcatccgaggccgtcggagaagggctgggggctgtctgcggcctgagatccgagagattattttttccaggtgagccggcctggccagcgggaagcccacaggcctgaggccgcccagttcccgcccatcctgcgcccgcccggtctgaccgatgtccttggccttgcgcggcaccaggcgccgctgcaaccagaccatcttgatggcgtccaggcggatctccacgaggttgctgaagagcgcgagcagcggcgccagcgggaaggcggccacgaagatggtggtgaagccgtactggatcactgcgcggtgggggtcaggctcaccggcgccccgcactcatgtccgcggacccccgccccgcattcgtctccgcgaacccccgccccgcagcgcccacgcactcatctccatgaactcgtcgaacaggctgaaggtgttgaccgggttcagaaggtagttgcgccgccagtccctgagctcggggtcccggggcaggtgcccggactcggaggcccgcagagagcggcacttgtgggtcacccacgggaccaggtactcgacgcagttgctgagcgtctgcttcaggcccatgatgatggccatctgcacgaagaggtccatcatgcagccgctggcgtggcactcttccagcttccacaagcccgccaggcgcgtggacttcccggggtggccgttgatctctgtcacccaggctggagcgcaatggtgcgatttcagttcactgcaacctctgcctcctgggttcaagtgattcttgtgcctcagcctcccgagtagctgggactacaggctcacaccaccacgcctggctagtagagacggggtttcttcatgttggccagtctggtcttgaactcctgacctcaggtgatctgcctgcctcagcctcccaaagtgctgggatttcaggcataagccactgcacctgcccaggatgaaggcgatgtagatgagagacgagaaatgggtgaagaactgcagtgtgaagaagcggatggtgaacctgctctctcgctccgagaaggtcctgggcatctcgaagtcacaaagcttcagggccacgcacctgttgatcttggtcatgatgatgatggtcacatagtgcaccagagccccggtcaccaccacggccgtggtcacctgctcctccaggaagggcacggccgagctgctgaagagcgcggaggccaggacgcggtagaccaccaggacgtgggccatgccgatcatgaggcagatcatgagcagggtcaggacgaggatgacggtgctgcgtaggtaggagtgctggtatggccggagcttgtagtcggggcagttaatgagctgaagtgccatttcctcctgttcctcgtcccacacgtacaggtcccagtgcaggaccacgcgggcgcgctgccgcttccagatctccaggaacaccgtggcccagagagccatgaagatggcgaacaccaccgtgccatcattgtcaaagaggtgggtgagcttggcaaaagtgcaggtttccgagagccgctggtacctgcggctgtggtcgccgaggggacacatgaggatgtcgtgggcctcacagatctccttgctgatctggctggcctcaaacagcgagaatccgctcagaaagactaagaggcccgtcagggcggccggcaccagcatgtaggtgtaccagcccagccagacgaagtacagggccaccttttccccaaagtagttcctgatttcatcaactggctgctcccggaacatgtgtctccaccgcgcccacgtcttcttcaggcgtccctcccccttgtgcagggggaacctggcctcaaagaccccgtccttcatcagatcctcgaaggtctcaccagccgaggtcttgttgttcatgacaacgaagttcacgattcggattctgagactcgtggtgaccgggatggtggtcggcgcggccagctcggcgtggggggcaggcccctcaggctccaggaggagagtgcggtacaggccaaagacactgttgtcagcacggatcccaaagaagacctgtttctggtcccggatcaccttaatgtggaagccctttctcctgagctcctccaggaactgttgctgccgcgcctgccgggggtctctctgggtgtgacgttgggccacgaggacatagtcccactgctcggaggcctcggtctcacaggtgctgatctccatcagcgggaagctgtccccttcgggctccaccaggatccggaggctctcttcgccctgcatgctggctgtggccggagttccagctggggtttggcggccaggagagtggctgccagcggcgggtgctcctacctgacttccgcgt

SEQ ID NO: 8942 - RNA, 2425 nt, Homo sapiens
  source 1..2425: mol_type = other RNA
accccactcctggtaccctcccacccaggctcaacccgcatccgaggccgtcggagaagggctgggggctgtctgcggcctgagatccgagagattattttttccaggtgagccggcctggccagcgggaagcccacaggcctgaggccgcccagttcccgcccatcctgcgcccgcccggtctgaccgatgtccttggccttgcgcggcaccaggcgccgctgcaaccagaccatcttgatggcgtccaggcggatctccacgaggttgctgaagagcgcgagcagcggcgccagcgggaaggcggccacgaagatggtggtgaagccgtactggatcactgcgcggtgggggtcaggctcaccggcgccccgcactcatgtccgcggacccccgccccgcattcgtctccgcgaacccccgccccgcagcgcccacgcactcatctccatgaactcgtcgaacaggctgaaggtgttgaccgggttcagaaggtagttgcgccgccagtccctgagctcggggtcccggggcaggtgcccggactcggaggcccgcagagagcggcacttgtgggtcacccacgggaccaggtactcgacgcagttgctgagcgtctgcttcaggcccatgatgatggccatctgcacgaagaggtccatcatgcagccgctggcgtggcactcttccagcttccacaagcccgccaggcgcgtggacttcccggggtggccgttgatctctgtcacccaggctggagcgcaatggtgcgatttcagttcactgcaacctctgcctcctgggttcaagtgattcttgtgcctcagcctcccgagtagctgggactacaggctcacaccaccacgcctggctagtagagacggggtttcttcatgttggccagtctggtcttgaactcctgacctcaggtgatctgcctgcctcagcctcccaaagtgctgggatttcaggcataagccactgcacctgcccaggatgaaggcgatgtagatgagagacgagaaatgggtgaagaactgcagtgtgaagaagcggatggtgaacctgctctctcgctccgagaaggtcctgggcatctctggaatgggaccggccctcacctctctccctgctcataggagaggccctgttgatcttggtcatgatgatgatggtcacatagtgcaccagagccccggtcaccaccacggccgtggtcacctgctcctccaggaagggcacggccgagctgctgaagagcgcggaggccaggacgcggtagaccaccaggacgtgggccatgccgatcatgaggcagatcatgagcagggtcaggacgaggatgacggtgctgcgtaggtaggagtgctggtatggccggagcttgtagtcggggcagttaatgagctgaagtgccatttcctcctgttcctcgtcccacacgtacaggtcccagtgcaggaccacgcgggcgcgctgccgcttccagatctccaggaacaccgtggcccagagagccatgaagatggcgaacaccaccgtgccatcattgtcaaagaggtgggtgagcttggcaaaagtgcaggtttccgagagccgctggtacctgcggctgtggtcgccgaggggacacatgaggatgtcgtgggcctcacagatctccttgctgatctggctggcctcaaacagcgagaatccgctcagaaagactaagaggcccgtcagggcggccggcaccagcatgtaggtgtaccagcccagccagacgaagtacagggccaccttttccccaaagtagttcctgatttcatcaactggctgctcccggaacatgtgtctccaccgcgcccacgtcttcttcaggcgtccctcccccttgtgcagggggaacctggcctcaaagaccccgtccttcatcagatcctcgaaggtctcaccagccgaggtcttgttgttcatgacaacgaagttcacgattcggattctgagactcgtggtgaccgggatggtggtcggcgcggccagctcggcgtggggggcaggcccctcaggctccaggaggagagtgcggtacaggccaaagacactgttgtcagcacggatcccaaagaagacctgtttctggtcccggatcaccttaatgtggaagccctttctcctgagctcctccaggaactgttgctgccgcgcctgccgggggtctctctgggtgtgacgttgggccacgaggacatagtcccactgctcggaggcctcggtctcacaggtgctgatctccatcagcgggaagctgtccccttcgggctccaccaggatccggaggctctcttcgccctgcatgctggctgtggccggagttccagctggggtttggcggccaggagagtggctgccagcggcgggtgctcctacctgacttccgcgt

SEQ ID NO: 8943 - RNA, 2154 nt, Homo sapiens
  source 1..2154: mol_type = other RNA
accccactcctggtaccctcccacccaggctcaacccgcatccgaggccgtcggagaagggctgggggctgtctgcggcctgagatccgagagattattttttccaggtgagccggcctggccagcgggaagcccacaggcctgaggccgcccagttcccgcccatcctgcgcccgcccggtctgaccgatgtccttggccttgcgcggcaccaggcgccgctgcaaccagaccatcttgatggcgtccaggcggatctccacgaggttgctgaagagcgcgagcagcggcgccagcgggaaggcggccacgaagatggtggtgaagccgtactggatcatcatctccatgaactcgtcgaacaggctgaaggtgttgaccgggttcagaaggtagttgcgccgccagtccctgagctcggggtcccggggcaggtgcccggactcggaggcccgcagagagcggcacttgtgggtcacccacgggaccaggtactcgacgcagttgctgagcgtctgcttcaggcccatgatgatggccatctgcacgaagaggtccatcatgcagccgctggcgtggcactcttccagcttccacaagcccgccaggcgcgtggacttcccggggtggccgttgatcctgcccaggatgaaggcgatgtagatgagagacgagaaatgggtgaagaactgcagtgtgaagaagcggatggtgaacctgctctctcgctccgagaaggtcctgggcatctcgaagtcacaaagcttcagggccacgcacctgttgatcttggtcatgatgatgatggtcacatagtgcaccagagccccggtcaccaccacggccgtggtcacctgctcctccaggaagggcacggccgagctgctgaagagcgcggaggccaggacgcggtagaccaccaggacgtgggccatgccgatcatgaggcagatcatgagcagggtcaggacgaggatgacggtgctgcgtaggtaggagtgctggtatggccggagcttgtagtcggggcagttaatgagctgaagtgccatttcctcctcagacacggcaggcatatgtgggccgtgcagggcatcgggcgccaacagcccctgctcgggtcggcctcagctgcgctgccagctccacctcacctgttcctcgtcccacacgtacaggtcccagtgcaggaccacgcgggcgcgctgccgcttccagatctccaggaacaccgtggcccagagagccatgaagatggcgaacaccaccgtgccatcattgtcaaagaggtgggtgagcttggcaaaagtgcaggtttccgagagccgctggtacctgcggctgtggtcgccgaggggacacatgaggatgtcgtgggcctcacagatctccttgctgatctggctggcctcaaacagcgagaatccgctcagaaagactaagaggcccgtcagggcggccggcaccagcatgtaggtgtaccagcccagccagacgaagtacagggccaccttttccccaaagtagttcctgatttcatcaactggctgctcccggaacatgtgtctccaccgcgcccacgtcttcttcaggcgtccctcccccttgtgcagggggaacctggcctcaaagaccccgtccttcatcagatcctcgaaggtctcaccagccgaggtcttgttgttcatgacaacgaagttcacgattcggattctgagactcgtggtgaccgggatggtggtcggcgcggccagctcggcgtggggggcaggcccctcaggctccaggaggagagtgcggtacaggccaaagacactgttgtcagcacggatcccaaagaagacctgtttctggtcccggatcaccttaatgtggaagccctttctcctgagctcctccaggaactgttgctgccgcgcctgccgggggtctctctgggtgtgacgttgggccacgaggacatagtcccactgctcggaggcctcggtctcacaggtgctgatctccatcagcgggaagctgtccccttcgggctccaccaggatccggaggctctcttcgccctgcatgctggctgtggccggagttccagctggggtttggcggccaggagagtggctgccagcggcgggtgctcctacctgacttccgcgt

SEQ ID NO: 8944 - RNA, 2062 nt, Homo sapiens
  source 1..2062: mol_type = other RNA
accccactcctggtaccctcccacccaggctcaacccgcatccgaggccgtcggagaagggctgggggctgtctgcggcctgagatccgagagattattttttccaggtgagccggcctggccagcgggaagcccacaggcctgaggccgcccagttcccgcccatcctgcgcccgcccggtctgaccgatgtccttggccttgcgcggcaccaggcgccgctgcaaccagaccatcttgatggcgtccaggcggatctccacgaggttgctgaagagcgcgagcagcggcgccagcgggaaggcggccacgaagatggtggtgaagccgtactggatcatcatctccatgaactcgtcgaacaggctgaaggtgttgaccgggttcagaaggtagttgcgccgccagtccctgagctcggggtcccggggcaggtgcccggactcggaggcccgcagagagcggcacttgtgggtcacccacgggaccaggtactcgacgcagttgctgagcgtctgcttcaggcccatgatgatggccatctgcacgaagaggtccatcatgcagccgctggcgtggcactcttccagcttccacaagcccgccaggcgcgtggacttcccggggtggccgttgatcctgcccaggatgaaggcgatgtagatgagagacgagaaatgggtgaagaactgcagtgtgaagaagcggatggtgaacctgctctctcgctccgagaaggtcctgggcatctcgaagtcacaaagcttcagggccacgcacctgttgatcttggtcatgatgatgatggtcacatagtgcaccagagccccggtcaccaccacggccgtggtcacctgctcctccaggaagggcacggccgagctgctgaagagcgcggaggccaggacgcggtagaccaccaggacgtgggccatgccgatcatgaggcagatcatgagcagggtcaggacgaggatgacggtgctgcgtaggtaggagtgctggtatggccggagcttgtagtcggggcagttaatgagctgaagtgccatttcctcctgttcctcgtcccacacgtacaggtcccagtgcaggaccacgcgggcgcgctgccgcttccagatctccaggaacaccgtggcccagagagccatgaagatggcgaacaccaccgtgccatcattgtcaaagaggtgggtgagcttggcaaaagtgcaggtttccgagagccgctggtacctgcggctgtggtcgccgaggggacacatgaggatgtcgtgggcctcacagatctccttgctgatctggctggcctcaaacagcgagaatccgctcagaaagactaagaggcccgtcagggcggccggcaccagcatgtaggtgtaccagcccagccagacgaagtacagggccaccttttccccaaagtagttcctgatttcatcaactggctgctcccggaacatgtgtctccaccgcgcccacgtcttcttcaggcgtccctccccctggcttgtgcagggggaacctggcctcaaagaccccgtccttcatcagatcctcgaaggtctcaccagccgaggtcttgttgttcatgacaacgaagttcacgattcggattctgagactcgtggtgaccgggatggtggtcggcgcggccagctcggcgtggggggcaggcccctcaggctccaggaggagagtgcggtacaggccaaagacactgttgtcagcacggatcccaaagaagacctgtttctggtcccggatcaccttaatgtggaagccctttctcctgagctcctccaggaactgttgctgccgcgcctgccgggggtctctctgggtgtgacgttgggccacgaggacatagtcccactgctcggaggcctcggtctcacaggtgctgatctccatcagcgggaagctgtccccttcgggctccaccaggatccggaggctctcttcgccctgcatgctggctgtggccggagttccagctggggtttggcggccaggagagtggctgccagcggcgggtgctcctacctgacttccgcgt

SEQ ID NO: 8945 - RNA, 2052 nt, Homo sapiens
  source 1..2052: mol_type = other RNA
accccactcctggtaccctcccacccaggctcaacccgcatccgaggccgtcggagaagggctgggggctgtctgcggcctgagatccgagagattattttttccaggtgagccggcctggccagcgggaagcccacaggcctgaggccgcccagttcccgcccatcctgcgcccgcccggtctgaccgatgtccttggccttgcgcggcaccaggcgccgctgcaaccagaccatcttgatggcgtccaggcggatctccacgaggttgctgaagagcgcgagcagcggcgccagcgggaaggcggccacgaagatggtggtgaagccgtactggatcatcatctccatgaactcgtcgaacaggctgaaggtgttgaccgggttcagaaggtagttgcgccgccagtccctgagctcggggtcccggggcaggtgcccggactcggaggcccgcagagagcggcacttgtgggtcacccacgggaccaggtactcgacgcagttgctgagcgtctgcttcaggcccatgatgatggccatctgcacgaagaggtccatcatgcagccgctggcgtggcactcttccagcttccacaagcccgccaggcgcgtggacttcccggggtggccgttgatcctgcccaggatgaaggcgatgtagatgagagacgagaaatgggtgaagaactgcagtgtgaagaagcggatggtgaacctgctctctcgctccgagaaggtcctgggcatctcgaagtcacaaagcttcagggccacgcacctgttgatcttggtcatgatgatgatggtcacatagtgcaccagagccccggtcaccaccacggccgtggtcacctgctcctccaggaagggcacggccgagctgctgaagagcgcggaggccaggacgcggtagaccaccaggacgtgggccatgccgatcatgaggcagatcatgagcagggtcaggacgaggatgacggtgctgcgtaggtaggagtgctggtatggccggagcttgtagtcggggcagttaatgagctgaagtgccatttcctcctgttcctcgtcccacacgtacaggtcccagtgcaggaccacgcgggcgcgctgccgcttccagatctccaggaacaccgtggcccagagagccatgaagatggcgaacaccaccgtgccatcattgtcaaagaggtgggtgagcttggcaaaagtgcaggtttccgagagccgctggtacctgcggctgtggtcgccgaggggacacatgaggatgtcgtgggcctcacagatctccttgctgatctggctggcctcaaacagcgagaatccgctcagaaagactaagaggcccgtcagggcggccggcaccagcatgtaggtgtaccagcccagccagacgaagtacagggccaccttttccccaaagtagttcctgatttcatcaactggctgctcccggaacatgtgtctccaccgcgcccacgtcttcttcaggcgtccctcccccttgtgcagggggaacctggcctcaaagaccccgtccttcatcagatcctcgaaggtctcaccagccgaggtcttgttgttcatgacaacgaagttcacgattcggattctcgtggtgaccgggatggtggtcggcgcggccagctcggcgtggggggcaggcccctcaggctccaggaggagagtgcggtacaggccaaagacactgttgtcagcacggatcccaaagaagacctgtttctggtcccggatcaccttaatgtggaagccctttctcctgagctcctccaggaactgttgctgccgcgcctgccgggggtctctctgggtgtgacgttgggccacgaggacatagtcccactgctcggaggcctcggtctcacaggtgctgatctccatcagcgggaagctgtccccttcgggctccaccaggatccggaggctctcttcgccctgcatgctggctgtggccggagttccagctggggtttggcggccaggagagtggctgccagcggcgggtgctcctacctgacttccgcgt

SEQ ID NO: 8946 - RNA, 2058 nt, Homo sapiens
  source 1..2058: mol_type = other RNA
accccactcctggtaccctcccacccaggctcaacccgcatccgaggccgtcggagaagggctgggggctgtctgcggcctgagatccgagagattattttttccaggtgagccggcctggccagcgggaagcccacaggcctgaggccgcccagttcccgcccatcctgcgcccgcccggtctgaccgatgtccttggccttgcgcggcaccaggcgccgctgcaaccagaccatcttgatggcgtccaggcggatctccacgaggttgctgaagagcgcgagcagcggcgccagcgggaaggcggccacgaagatggtggtgaagccgtactggatcatcatctccatgaactcgtcgaacaggctgaaggtgttgaccgggttcagaaggtagttgcgccgccagtccctgagctcggggtcccggggcaggtgcccggactcggaggcccgcagagagcggcacttgtgggtcacccacgggaccaggtactcgacgcagttgctgagcgtctgcttcaggcccatgatgatggccatctgcacgaagaggtccatcatgcagccgctggcgtggcactcttccagcttccacaagcccgccaggcgcgtggacttcccggggtggccgttgatcctgcccaggatgaaggcgatgtagatgagagacgagaaatgggtgaagaactgcagtgtgaagaagcggatggtgaacctgctctctcgctccgagaaggtcctgggcatctcgaagtcacaaagcttcagggccacgcacctgttgatcttggtcatgatgatgatggtcacatagtgcaccagagccccggtcaccaccacggccgtggtcacctgctcctccaggaagggcacggccgagctgctgaagagcgcggaggccaggacgcggtagaccaccaggacgtgggccatgccgatcatgaggcagatcatgagcagggtcaggacgaggatgacggtgctgcgtaggtaggagtgctggtatggccggagcttgtagtcggggcagttaatgagctgaagtgccatttcctcctgttcctcgtcccacacgtacaggtcccagtgcaggaccacgcgggcgcgctgccgcttccagatctccaggaacaccgtggcccagagagccatgaagatggcgaacaccaccgtgccatcattgtcaaagaggtgggtgagcttggcaaaagtgcaggtttccgagagccgctggtacctgcggctgtggtcgccgaggggacacatgaggatgtcgtgggcctcacagatctccttgctgatctggctggcctcaaacagcgagaatccgctcagaaagactaagaggcccgtcagggcggccggcaccagcatgtaggtgtaccagcccagccagacgaagtacagggccaccttttccccaaagtagttcctgatttcatcaactggctgctcccggaacatgtgtctccaccgcgcccacgtcttcttcaggcgtccctcccccttgtgcagggggaacctggcctcaaagaccccgtccttcatcagatcctcgaaggtctcaccagccgaggtcttgttgttcatgacaacgaagttcacgattcggattctgagactcgtggtgaccgggatggtggtcggcgcggccagctcggcgtggggggcaggcccctcaggctccaggaggagagtgcggtacaggccaaagacactgttgtcagcacggatcccaaagaagacctgtttctggtcccggatcaccttaatgtggaagccctttctcctgagctcctccaggaactgttgctgccgcgcctgccgggggtctctctgggtgtgacgttgggccacgaggacatagtcccactgctcggaggcctcggtctcacaggtgctgatctccatcagcgggaagctgtccccttcgggctccaccaggatccggaggctctcttcgccctgcatgctggctgtggccggagttccagctggggtttggcggccaggagagtggctgccagcggcgggtgctcctacctgacttccgcgt

SEQ ID NO: 8947 - RNA, 840 nt, Homo sapiens
  source 1..840: mol_type = other RNA
accccactcctggtaccctcccacccaggctcaacccgcatccgaggccgtcggagaagggctgggggctgtctgcggcctgagatccgagagattattttttccaggtgagccggcctggccagcgggaagcccacaggcctgaggccgcccagttcccgcccatcctgcgcccgcccggtctgaccgatgtccttggccttgcgcggcaccaggcgccgctgcaaccagaccatcttgatggcgtccaggcggatctccacgaggttgctgaagagcgcgagcagcggcgccagcgggaaggcggccacgaagatggtggtgaagccgtactggatcatcatctccatgaactcgtcgaacaggctgaaggtgttgaccgggttcagaaggtagttgcgccgccagtccctgagctcggggtcccggggcaggtgcccggactcggaggcccgcagagagcggcacttgtgggtcacccacgggaccaggtactcgacgcagttgctgagcgtctgcttcaggcccatgatgatggccatctgcacgaagaggtccatcatgcagccgctggcgtggcactcttccagcttccacaagcccgccaggcgcgtggacttcccggggtggccgttgatcctgcccaggatgaaggcgatgtagatgagagacgagaaatgggtgaagaactgcagtgtgaagaagcggatggtgaacctgctctctcgctccgagaaggtcctgggcatctctggaatgggaccggccctcacctctctccctgctcataggagaggcccgaagtcacaaagcttcagggccacgcacctgttgatctgc

SEQ ID NO: 8948 - RNA, 2077 nt, Homo sapiens
  source 1..2077: mol_type = other RNA
accccactcctggtaccctcccacccaggctcaacccgcatccgaggccgtcggagaagggctgggggctgtctgcggcctgagatccgagagattattttttccaggtgagccggcctggccagcgggaagcccacaggcctgaggccgcccagttcccgcccatcctgcgcccgcccggtctgaccgatgtccttggccttgcgcggcaccaggcgccgctgcaaccagaccatcttgatggcgtccaggcggatctccacgaggttgctgaagagcgcgagcagcggcgccagcgggaaggcggccacgaagatggtggtgaagccgtactggatcatcatctccatgaactcgtcgaacaggctgaaggtgttgaccgggttcagaaggtagttgcgccgccagtccctgagctcggggtcccggggcaggtgcccggactcggaggcccgcagagagcggcacttgtgggtcacccacgggaccaggtactcgacgcagttgctgagcgtctgcttcaggcccatgatgatggccatctgcacgaagaggtccatcatgcagccgctggcgtggcactcttccagcttccacaagcccgccaggcgcgtggacttcccggggtggccgttgatcctgcccaggatgaaggcgatgtagatgagagacgagaaatgggtgaagaactgcagtgtgaagaagcggatggtgaacctgctctctcgctccgagaaggtcctgggcatctctggaatgggaccggccctcacctctctccctgctcataggagaggccctgttgatcttggtcatgatgatgatggtcacatagtgcaccagagccccggtcaccaccacggccgtggtcacctgctcctccaggaagggcacggccgagctgctgaagagcgcggaggccaggacgcggtagaccaccaggacgtgggccatgccgatcatgaggcagatcatgagcagggtcaggacgaggatgacggtgctgcgtaggtaggagtgctggtatggccggagcttgtagtcggggcagttaatgagctgaagtgccatttcctcctgttcctcgtcccacacgtacaggtcccagtgcaggaccacgcgggcgcgctgccgcttccagatctccaggaacaccgtggcccagagagccatgaagatggcgaacaccaccgtgccatcattgtcaaagaggtgggtgagcttggcaaaagtgcaggtttccgagagccgctggtacctgcggctgtggtcgccgaggggacacatgaggatgtcgtgggcctcacagatctccttgctgatctggctggcctcaaacagcgagaatccgctcagaaagactaagaggcccgtcagggcggccggcaccagcatgtaggtgtaccagcccagccagacgaagtacagggccaccttttccccaaagtagttcctgatttcatcaactggctgctcccggaacatgtgtctccaccgcgcccacgtcttcttcaggcgtccctcccccttgtgcagggggaacctggcctcaaagaccccgtccttcatcagatcctcgaaggtctcaccagccgaggtcttgttgttcatgacaacgaagttcacgattcggattctgagactcgtggtgaccgggatggtggtcggcgcggccagctcggcgtggggggcaggcccctcaggctccaggaggagagtgcggtacaggccaaagacactgttgtcagcacggatcccaaagaagacctgtttctggtcccggatcaccttaatgtggaagccctttctcctgagctcctccaggaactgttgctgccgcgcctgccgggggtctctctgggtgtgacgttgggccacgaggacatagtcccactgctcggaggcctcggtctcacaggtgctgatctccatcagcgggaagctgtccccttcgggctccaccaggatccggaggctctcttcgccctgcatgctggctgtggccggagttccagctggggtttggcggccaggagagtggctgccagcggcgggtgctcctacctgacttccgcgt

SEQ ID NO: 8949 - RNA, 953 nt, Homo sapiens
  source 1..953: mol_type = other RNA
accccactcctggtaccctcccacccaggctcaacccgcatccgaggccgtcggagaagggctgggggctgtctgcggcctgagatccgagagattattttttccaggtgagccggcctggccagcgggaagcccacaggcctgaggccgcccagttcccgcccatcctgcgcccgcccggtctgaccgatgtccttggccttgcgcggcaccaggcgccgctgcaaccagaccatcttgatggcgtccaggcggatctccacgaggttgctgaagagcgcgagcagcggcgccagcgggaaggcggccacgaagatggtggtgaagccgtactggatcatcatctccatgaactcgtcgaacaggctgaaggtgttgaccgggttcagaaggtagttgcgccgccagtccctgagctcggggtcccggggcaggtgcccggactcggaggcccgcagagagcggcacttgtgggtcacccacgggaccaggtactcgacgcagttgctgagcgtctgcttcaggcccatgatgatggccatctgcacgaagaggtccatcatgcagccgctggcgtggcactcttccagcttccacaagcccgccaggcgcgtggacttcccggggtggccgttgatcctgcccaggatgaaggcgatgtagatgagagacgagaaatgggtgaagaactgcagtgtgaagaagcggatggtgaacctgctctctcgctccgagaaggtcctgggcatctctgttgatcttggtcatgatgatgatggtcacatagtgcaccagagccccggtcaccaccacggccgtggtcacctgctcctccaggaagggcacggccgagctgctgaagagcgcggaggccaggacgcggtagaccaccaggacgtgggccatgccgatcatgaggcagatcatgagcagggtcaggacgaggatgacgg

SEQ ID NO: 8950 - RNA, 2029 nt, Homo sapiens
  source 1..2029: mol_type = other RNA
accccactcctggtaccctcccacccaggctcaacccgcatccgaggccgtcggagaagggctgggggctgtctgcggcctgagatccgagagattattttttccaggtgagccggcctggccagcgggaagcccacaggcctgaggccgcccagttcccgcccatcctgcgcccgcccggtctgaccgatgtccttggccttgcgcggcaccaggcgccgctgcaaccagaccatcttgatggcgtccaggcggatctccacgaggttgctgaagagcgcgagcagcggcgccagcgggaaggcggccacgaagatggtggtgaagccgtactggatcatcatctccatgaactcgtcgaacaggctgaaggtgttgaccgggttcagaaggtagttgcgccgccagtccctgagctcggggtcccggggcaggtgcccggactcggaggcccgcagagagcggcacttgtgggtcacccacgggaccaggtactcgacgcagttgctgagcgtctgcttcaggcccatgatgatggccatctgcacgaagaggtccatcatgcagccgctggcgtggcactcttccagcttccacaagcccgccaggcgcgtggacttcccggggtggccgttgatcctgcccaggatgaaggcgatgtagatgagagacgagaaatgggtgaagaactgcagtgtgaagaagcggatggtgaacctgctctctcgctccgagaaggtcctgggcatctctgttgatcttggtcatgatgatgatggtcacatagtgcaccagagccccggtcaccaccacggccgtggtcacctgctcctccaggaagggcacggccgagctgctgaagagcgcggaggccaggacgcggtagaccaccaggacgtgggccatgccgatcatgaggcagatcatgagcagggtcaggacgaggatgacggtgctgcgtaggtaggagtgctggtatggccggagcttgtagtcggggcagttaatgagctgaagtgccatttcctcctgttcctcgtcccacacgtacaggtcccagtgcaggaccacgcgggcgcgctgccgcttccagatctccaggaacaccgtggcccagagagccatgaagatggcgaacaccaccgtgccatcattgtcaaagaggtgggtgagcttggcaaaagtgcaggtttccgagagccgctggtacctgcggctgtggtcgccgaggggacacatgaggatgtcgtgggcctcacagatctccttgctgatctggctggcctcaaacagcgagaatccgctcagaaagactaagaggcccgtcagggcggccggcaccagcatgtaggtgtaccagcccagccagacgaagtacagggccaccttttccccaaagtagttcctgatttcatcaactggctgctcccggaacatgtgtctccaccgcgcccacgtcttcttcaggcgtccctcccccttgtgcagggggaacctggcctcaaagaccccgtccttcatcagatcctcgaaggtctcaccagccgaggtcttgttgttcatgacaacgaagttcacgattcggattctgagactcgtggtgaccgggatggtggtcggcgcggccagctcggcgtggggggcaggcccctcaggctccaggaggagagtgcggtacaggccaaagacactgttgtcagcacggatcccaaagaagacctgtttctggtcccggatcaccttaatgtggaagccctttctcctgagctcctccaggaactgttgctgccgcgcctgccgggggtctctctgggtgtgacgttgggccacgaggacatagtcccactgctcggaggcctcggtctcacaggtgctgatctccatcagcgggaagctgtccccttcgggctccaccaggatccggaggctctcttcgccctgcatgctggctgtggccggagttccagctggggtttggcggccaggagagtggctgccagcggcgggtgctcctacctgacttccgcgt

SEQ ID NO: 8951 - RNA, 2188 nt, Homo sapiens
  source 1..2188: mol_type = other RNA
accccactcctggtaccctcccacccaggctcaacccgcatccgaggccgtcggagaagggctgggggctgtctgcggcctgagatccgagagattattttttccaggtgagccggcctggccagcgggaagcccacaggcctgaggccgcccagttcccgcccatcctgcgcccgcccggtctgaccgatgtccttggccttgcgcggcaccaggcgccgctgcaaccagaccatcttgatggcgtccaggcggatctccacgaggttgctgaagagcgcgagcagcggcgccagcgggaaggcggccacgaagatggtggtgaagccgtactggatcatcatctccatgaactcgtcgaacaggctgaaggtgttgaccgggttcagaaggtagttgcgccgccagtccctgagctcggggtcccggggcaggtgcccggactcggaggcccgcagagagcggcacttgtgggtcacccacgggaccaggtactcgacgcagttgctgagcgtctgcttcaggcccatgatgatggccatctgcacgaagaggtccatcatgcagccgctggcgtggcactcttccagcttccacaagcccgccaggcgcgtggacttcccggggtggccgttgatcctggaaaatcaaaataaaacaactgaaagcctgggtggataaatcaatcgagtgctcaagtggatacaaaacgagcatccagcagaactggcttttccgtgtgcggcaaagctgcccaggatgaaggcgatgtagatgagagacgagaaatgggtgaagaactgcagtgtgaagaagcggatggtgaacctgctctctcgctccgagaaggtcctgggcatctctggaatgggaccggccctcacctctctccctgctcataggagaggccctgttgatcttggtcatgatgatgatggtcacatagtgcaccagagccccggtcaccaccacggccgtggtcacctgctcctccaggaagggcacggccgagctgctgaagagcgcggaggccaggacgcggtagaccaccaggacgtgggccatgccgatcatgaggcagatcatgagcagggtcaggacgaggatgacggtgctgcgtaggtaggagtgctggtatggccggagcttgtagtcggggcagttaatgagctgaagtgccatttcctcctgttcctcgtcccacacgtacaggtcccagtgcaggaccacgcgggcgcgctgccgcttccagatctccaggaacaccgtggcccagagagccatgaagatggcgaacaccaccgtgccatcattgtcaaagaggtgggtgagcttggcaaaagtgcaggtttccgagagccgctggtacctgcggctgtggtcgccgaggggacacatgaggatgtcgtgggcctcacagatctccttgctgatctggctggcctcaaacagcgagaatccgctcagaaagactaagaggcccgtcagggcggccggcaccagcatgtaggtgtaccagcccagccagacgaagtacagggccaccttttccccaaagtagttcctgatttcatcaactggctgctcccggaacatgtgtctccaccgcgcccacgtcttcttcaggcgtccctcccccttgtgcagggggaacctggcctcaaagaccccgtccttcatcagatcctcgaaggtctcaccagccgaggtcttgttgttcatgacaacgaagttcacgattcggattctgagactcgtggtgaccgggatggtggtcggcgcggccagctcggcgtggggggcaggcccctcaggctccaggaggagagtgcggtacaggccaaagacactgttgtcagcacggatcccaaagaagacctgtttctggtcccggatcaccttaatgtggaagccctttctcctgagctcctccaggaactgttgctgccgcgcctgccgggggtctctctgggtgtgacgttgggccacgaggacatagtcccactgctcggaggcctcggtctcacaggtgctgatctccatcagcgggaagctgtccccttcgggctccaccaggatccggaggctctcttcgccctgcatgctggctgtggccggagttccagctggggtttggcggccaggagagtggctgccagcggcgggtgctcctacctgacttccgcgt

SEQ ID NO: 8952 - RNA, 2140 nt, Homo sapiens
  source 1..2140: mol_type = other RNA
accccactcctggtaccctcccacccaggctcaacccgcatccgaggccgtcggagaagggctgggggctgtctgcggcctgagatccgagagattattttttccaggtgagccggcctggccagcgggaagcccacaggcctgaggccgcccagttcccgcccatcctgcgcccgcccggtctgaccgatgtccttggccttgcgcggcaccaggcgccgctgcaaccagaccatcttgatggcgtccaggcggatctccacgaggttgctgaagagcgcgagcagcggcgccagcgggaaggcggccacgaagatggtggtgaagccgtactggatcatcatctccatgaactcgtcgaacaggctgaaggtgttgaccgggttcagaaggtagttgcgccgccagtccctgagctcggggtcccggggcaggtgcccggactcggaggcccgcagagagcggcacttgtgggtcacccacgggaccaggtactcgacgcagttgctgagcgtctgcttcaggcccatgatgatggccatctgcacgaagaggtccatcatgcagccgctggcgtggcactcttccagcttccacaagcccgccaggcgcgtggacttcccggggtggccgttgatcctggaaaatcaaaataaaacaactgaaagcctgggtggataaatcaatcgagtgctcaagtggatacaaaacgagcatccagcagaactggcttttccgtgtgcggcaaagctgcccaggatgaaggcgatgtagatgagagacgagaaatgggtgaagaactgcagtgtgaagaagcggatggtgaacctgctctctcgctccgagaaggtcctgggcatctctgttgatcttggtcatgatgatgatggtcacatagtgcaccagagccccggtcaccaccacggccgtggtcacctgctcctccaggaagggcacggccgagctgctgaagagcgcggaggccaggacgcggtagaccaccaggacgtgggccatgccgatcatgaggcagatcatgagcagggtcaggacgaggatgacggtgctgcgtaggtaggagtgctggtatggccggagcttgtagtcggggcagttaatgagctgaagtgccatttcctcctgttcctcgtcccacacgtacaggtcccagtgcaggaccacgcgggcgcgctgccgcttccagatctccaggaacaccgtggcccagagagccatgaagatggcgaacaccaccgtgccatcattgtcaaagaggtgggtgagcttggcaaaagtgcaggtttccgagagccgctggtacctgcggctgtggtcgccgaggggacacatgaggatgtcgtgggcctcacagatctccttgctgatctggctggcctcaaacagcgagaatccgctcagaaagactaagaggcccgtcagggcggccggcaccagcatgtaggtgtaccagcccagccagacgaagtacagggccaccttttccccaaagtagttcctgatttcatcaactggctgctcccggaacatgtgtctccaccgcgcccacgtcttcttcaggcgtccctcccccttgtgcagggggaacctggcctcaaagaccccgtccttcatcagatcctcgaaggtctcaccagccgaggtcttgttgttcatgacaacgaagttcacgattcggattctgagactcgtggtgaccgggatggtggtcggcgcggccagctcggcgtggggggcaggcccctcaggctccaggaggagagtgcggtacaggccaaagacactgttgtcagcacggatcccaaagaagacctgtttctggtcccggatcaccttaatgtggaagccctttctcctgagctcctccaggaactgttgctgccgcgcctgccgggggtctctctgggtgtgacgttgggccacgaggacatagtcccactgctcggaggcctcggtctcacaggtgctgatctccatcagcgggaagctgtccccttcgggctccaccaggatccggaggctctcttcgccctgcatgctggctgtggccggagttccagctggggtttggcggccaggagagtggctgccagcggcgggtgctcctacctgacttccgcgt

SEQ ID NO: 8953 - RNA, 3163 nt, Homo sapiens
  source 1..3163: mol_type = other RNA
acccgcccgtctccccacagctgccccaccccccgcccctggcaggaaatgccacactggggagggtctccagtctcaggggcgcggggctgcctgtcctccaccttcggattccaggcagttgtgacaacaccagctatcggcagagctattaatagtgtttcagggagtgacagggagagggctctgggggctggaagtccggccctggggcagggtgttccgcttacagctagtaccaagtggagggggcagggcccctgagtcaggaccctgagtcccccacgtatatggcagggcacagcatggggagggctgtaacagagaggcctcccatccaaagggggatggagacctggacaggaggtggccggggatacaacccccagcaccaccagggcttggagaggccacccaggcagaaggatgtggtgactggggtcttcagcaaccgcatttctggggctcccccctcccattcctgtccctgcgtcttcagcaccaatgtcgggagaggccacggggccacactgggtcacagttccaagggctcctccacaggcaccgactggagctgggtcagaaccttggcctcagcttccaacccctcgtcaacctcaccccctgcggtggcccccaggagcagcccctcagggtcggggtctggcagcctcagcacggtgtggggggcctgtgtccccagccccttttccgcttccagcagcccctctgttcctgcgcttagttccagccctgctgaccagacaggcacggccgcgggtgacaacatcagcccctctggtgggggcgccgggaagttgggcaggaggccaggggagtcaggggagaagggcaggctggtgctggaggtggtggcagcggcggggggtggctgctgtgcagaaagggtgcctagggcgtgagcctctgggagagcagggctgggggccaccgggaggcctccctcaggcacggagatggccgtctctggcttcagtggcagggccaggccgggggctggcggcaggacctgggagacgagcatgctggtggggaaggtggcggtgaggatgatcttgccctgctgcagggccacacccgtcacgatggggctgccagacacagggttggccaggaggaagtttcctggggcagtggccgaaggcagctgcagggcagtcacgcccaccccggagttgatgaggtgcacattggcagggcctgctgcagctgccaccttcacagggctgcctggcccggctgccaacagctgcaggggccccacagcctggggcagggtcaccacctgtgaggtgggtactacctggggcaggttcaatagtggggaggtggggctcaggcccgtgggataccccgggggtggggagagcggtaccacttgtggggcagccacagcaggcactggccccgggggcagaggaaaggtggcagccgtcggggggccaggcaccacttgggccaggggccccaggacctcctctccaagggctggtcccggagcagccacctgggcccctttggtctcaggggcctccgactgagcctcctccagccgcacctcccctgtctgagggtccaggaccagagaggtcttggtctcgctggccccctgagggctgggctgcggtggaggggcacccccgcccccagtgagcagcagcgggcccaggctggaggcctcgcccagggccaggccgttgatgatgacggggcccccgttgaggagcactgctggggagccgctggctgccaggaagctcccgttcaccaggatggaggaggaagccgggcaaggcgcgggagggccggtccctgccaggaatatggagccctgggcagcggcctcggcggacactggggccgcccctctctccaggtcctcaggacttcggctggactcgtcctcagtcgtgggattcccatcagactcgctcttgcagggcgcgccgcctccggccccggtccggtcgcgctgtcgccggttcttgaaccagttgctgacctgcgtgagcgacaggccggtgagtgtggccaggcggcgcttctcgtccggcgtggggtagcggttgccgcggtagcaggccttgagcgctgcgcgggagcgctccttgaagcagtagactgtctcctcgccgtcccagatggtcttgggcagcgggaacttcttgcgcagtcgatacttgtccactgcgccaagcgcgcggccgcgggcccgctcggcctcatggtagcgcgcgcgcaggtagaggtcctgcaggaaggcgtggtgggcggcggggaaggggcggctctcgagtagccggtagagctcggcgtactcgccccgctggaaggccaccagggcccgcgcgcgcaacaccgggtcgctgccacgtaggcgctcggccgggggcagtgcgcccaggaagcggctcaagcggccggcgtggcccgcctggagcagcgcctcgcagacgcacgccacctgctcgggcgagaagcggaggcccgtgggcggttcggaagcggcctcggggggcgacccggggacgcccggggatcccgggccctcagctcccgcagccgctgcgcccgccccggccccggccgccgccgccgcctcaccctcggccgcctgcaaagtctgcaagagctggcgcgcttcctcctcctcctcttcggtcgccgccgccgccgccaccgcctcccccccagccgccggccccgcgctcggctccgcaggcaaggtagccatgttttgcaactttgggaagttcctccctccctctcttcctccctcgggctttccccagcctcctcccccacctgtccccccttttcgcccccactccccgctcttctcgatcttctttctggccgaccctgcgccccacgccgggaaggcgagatccagctctccactcgggtctctgtccccttgtgtgtgtccgtccccctcccgtctgtctgtgattctccctttgttttccctccgcctctggccgcgctttctgcctccccccagcgtgtgcttctggctcagggcctcagtttccccatcgggacaacgcagaaggtaacgggccgtccaggaggactaagggcgcgaagcctccgccccgagactgagcttctgcacgcctccgtctccagggtcctctgc

SEQ ID NO: 8954 - RNA, 3121 nt, Homo sapiens
  source 1..3121: mol_type = other RNA
accctttttctctttcccagaactgaacaccagatggtagctttttaaccgtagctcaaaggtcattttaaatccacacataagctaaagagatcccttctgagatgaaggacaaagaataactttaaaagctaggtgaaaaaagaggcacttaaaggaaagatgtgttccaactctcccatgcgagtctcctgctgtgagttggccccgggaggaccagcgctgccccttgcacgccttcagcaccttgagtacacctgcggcttacacatgcgcatggtgagcctcttgctcagctcccctagcagccagatggcaaagcgagtgaaaatttatgtcattctttttagaattaaaaaaaaaacaaatcaaacaaaccagaactaaaatttcacacacacaaaatgaatgctactcagtttcattccttcctcatgctagtttttaaatgatacttggttcttcaggaaggatgacctgtggctttacccccaagaccttgtatccaattactagacaattattcacagcaccatgcacattaaagcagacggaaaagaaggcaacaagctaagggaaaaatcaaggaccaactgcctgagaaaatggcaggtacctggcccagagattagaaaagaaacaagttctcaaaaggaaatggccaagatgatagccaaagaccacagcccgagtggaagccaagttaacaagcccagaggatgcaggttttctctgcctggctcttctctggcctccctcgggagcttgtgttcatgttacatggcatttacaccacatacttagggtctacaattccccatgaagaagtcaaagagatatttaaaaccattaataagcataagagagtttcaaaactgccagaatgaagaactttggccaccacaagtttttccgtttgaaacattcttggtgccataatttctaagagcaacaacaaagagcacgaccacgacacacacgtaagtcttttgacaaaccaactctaaccactgctggcaccatgaggatgagaaagaaatcactaaccaagagttgctgggctgcttaaccttccttcaaagccaaagggtaggtttgagttatctgtgcaacaagatggcaagcactgctgccatcagacccagctactactcagttagacacatcttgaaaacactaagttaaacatctaggtttaagtataacctgcaagattcccaaggttagccttctcagcttcccctaaatttgtggttgttgctgttgctagatgtaaaaattttttaatttcatttttctttatgttgatgatgttttaatttctagaatattgtatgacatggaactattcagaattcctttaaaaaggaatctgtcttgattaataacattattaaggtactttcaggctttcccttaactccatcgagaaggaagagggagtatgtgagtacatgtgcatgtaatgggtcaggaggaacagaagcaaagaaggaagcacgtgggaaagtgagatgtccataaactgaaaaaccaatttacagaaaggcatctgatgtattttctaaataaggccttgatcagggtaaccaatcctctttgtagcacattctacactgcccataaataaaggagtctctttaaattaacatttccagtatcaatgaacagtccagaaatcctcatttcaagcgttcgatgagtccctgtgtgagtccaaggtgcagaagttgtgttcgggagaggtttgcaaggttagggaaggccgcaagcagcttctcccatgccagttccagcaggctaggtaccaccagccagatcttaaacaatgacccagtccgtttgttttcatggatgttcaccactcctccatgaatgtacatgcaaccagctggtgtaacagctgcacagtgaaaataaactggctctggcatggtagctgggagcttcacccattggaaagtctgcagattcaacttccagatatctcccaggatcacctctccattatagcccccacaaataaatacatcattttttatttgaacacaactgtgacaccttcgggctgcaggaaagcctattttttcatggggttttgttgcaatttcctcccaggcattcgtttcaaggttgtatgcatggatcttgtttaaggaatatgctgtccaggaagtaccacctcccaagatgtaaatcctctgcccgtcatgtgcaatttcatgtcggtatctctcttctggtagatcacaggataggttgtttggtttcagttgtgtccactctctggtattgagatctaacttgtgcaggtctgtgctgtaaatatagccggttgtacctccaaagacataaagggagccattgatgatggccatagcctgtccatatatacgactgggtttcttcccccgacagctgagcaaagcccatctcttatacttcacattacacacatggacgtcattgccgttgctctctccaaatgggatgcccgtacctccaaatactaacaggttgtttccatgcagcacaagtgacatagatgccaattcccggggcatgtagccatctgtgcccatctggtgccatactcctgtagcaaaatgatacctccagagttccctgaagagaggatagtcttcattatcaggccctcccgattcatcataatctgggttataacctccaaacacatataggttggtattatctgccacacaacgatgtccacttcgtgctggtggaggtctgtggcctctcaaaaacctgttagggatccttatgatgggacaggactgaatgaagcgcctcctaactgggtcccatcgtattttcttcttacctggcaggtgcggccgcccggagagttgcacgaagcggttgagctggccagtcccccgacccccgctgcccccactgcccccgccggccccgctacctccgccaccagcgccggcggcgcctcctcccctccggcggttcctgtcccagccctgggcggccgacatgacccgctaacgattgccgcagcccggtcccgtcagcgcctgacccagcggaaccagcggagcctccttcctgggctcctccagagacccaggagacaggggaagggggc

SEQ ID NO: 8955 - RNA, 3036 nt, Homo sapiens
  source 1..3036: mol_type = other RNA
accctttttctctttcccagaactgaacaccagatggtagctttttaaccgtagctcaaaggtcattttaaatccacacataagctaaagagatcccttctgagatgaaggacaaagaataactttaaaagctaggtgaaaaaagaggcacttaaaggaaagatgtgttccaactctcccatgcgagtctcctgctgtgagttggccccgggaggaccagcgctgccccttgcacgccttcagcaccttgagtacacctgcggcttacacatgcgcatggtgagcctcttgctcagctcccctagcagccagatggcaaagcgagtgaaaatttatgtcattctttttagaattaaaaaaaaaacaaatcaaacaaaccagaactaaaatttcacacacacaaaatgaatgctactcagtttcattccttcctcatgctagtttttaaatgatacttggttcttcaggaaggatgacctgtggctttacccccaagaccttgtatccaattactagacaattattcacagcaccatgcacattaaagcagacggaaaagaaggcaacaagctaagggaaaaatcaaggaccaactgcctgagaaaatggcaggtacctggcccagagattagaaaagaaacaagttctcaaaaggaaatggccaagatgatagccaaagaccacagcccgagtggaagccaagttaacaagcccagaggatgcaggttttctctgcctggctcttctctggcctccctcgggagcttgtgttcatgttacatggcatttacaccacatacttagggtctacaattccccatgaagaagtcaaagagatatttaaaaccattaataagcataagagagtttcaaaactgccagaatgaagaactttggccaccacaagtttttccgtttgaaacattcttggtgccataatttctaagagcaacaacaaagagcacgaccacgacacacacgtaagtcttttgacaaaccaactctaaccactgctggcaccatgaggatgagaaagaaatcactaaccaagagttgctgggctgcttaaccttccttcaaagccaaagggtaggtttgagttatctgtgcaacaagatggcaagcactgctgccatcagacccagctactactcagttagacacatcttgaaaacactaagttaaacatctaggtttaagtataacctgcaagattcccaaggttagccttctcagcttcccctaaatttgtggttgttgctgttgctagatgtaaaaattttttaatttcatttttctttatgttgatgatgttttaatttctagaatattgtatgacatggaactattcagaattcctttaaaaaggaatctgtcttgattaataacattattaaggtactttcaggctttcccttaactccatcgagaaggaagagggagtatgtgagtacatgtgcatgtaatgggtcaggaggaacagaagcaaagaaggaagcacgtgggaaagtgagatgtccataaactgaaaaaccaatttacagaaaggcatctgatgtattttctaaataaggccttgatcagggtaaccaatcctctttgtagcacattctacactgcccataaataaaggagtctctttaaattaacatttccagtatcaatgaacagtccagaaatcctcatttcaagcgttcgatgagtccctgtgtgagtccaaggtgcagaagttgtgttcgggagaggtttgcaaggttagggaaggccgcaagcagcttctcccatgccagttccagcaggctaggtaccaccagccagatcttaaacaatgacccagtccgtttgttttcatggatgttcaccactcctccatgaatgtacatgcaaccagctggtgtaacagctgcacagtgaaaataaactggctctggcatggtagctgggagcttcacccattggaaagtctgcagattcaacttccagatatctcccaggatcacctctccattatagcccccacaaataaatacatcattttttatttgaacacaactgtgacaccttcgggctgcaggaaagcctattttttcatggggttttgttgcaatttcctcccaggcattcgtttcaaggttgtatgcatggatcttgtttaaggaatatgctgtccaggaagtaccacctcccaagatgtaaatcctctgcccgtcatgtgcaatttcatgtcggtatctctcttctggtagatcacaggataggttgtttggtttcagttgtgtccactctctggtattgagatctaacttgtgcaggtctgtgctgtaaatatagccggttgtacctccaaagacataaagggagccattgatgatggccatagcctgtccatatatacgactgggtttcttcccccgacagctgagcaaagcccatctcttatacttcacattacacacatggacgtcattgccgttgctctctccaaatgggatgcccgtacctccaaatactaacaggttgtttccatgcagcacaagtgacatagatgccaattcccggggcatgtagccatctgtgcccatctggtgccatactcctgtagcaaaatgatacctccagagttccctgaagagaggatagtcttcattatcaggccctcccgattcatcataatctgggttataacctccaaacacatataggttggtattatctgccacacaacgatgtccacttcgtgctggtggaggtctgtggcctggcaggtgcggccgcccggagagttgcacgaagcggttgagctggccagtcccccgacccccgctgcccccactgcccccgccggccccgctacctccgccaccagcgccggcggcgcctcctcccctccggcggttcctgtcccagccctgggcggccgacatgacccgctaacgattgccgcagcccggtcccgtcagcgcctgacccagcggaaccagcggagcctccttcctgggctcctccagagacccaggagacaggggaagggggcag

SEQ ID NO: 8956 - RNA, 7049 nt, Homo sapiens
  source 1..7049: mol_type = other RNA
accctttttctctttcccagagatgctaagtttgtatgtagctcaactttaattcgactagtttctagaaaagctggaacagtatctaccttaggttagggaaggacttgttcactactgtctccctagcatctagaactgtgtctgacatatattgggcacccagtatttgcagaataaatgaataaaatgagaagatgaaaatttcttaaagagtaagtatttacaggggacaagtatgcttttaactataacttttaactataacagctatcagtactccaattatccggagtcagatgtccaattccaaactgccaatactttatattagtttttcttctttccacattgcttacacagaataatcttattaggtaaagtctccttcattttaaattttttttcaaagcacacatgtgcattcatatgttaaatataatttttgacagaacattaaacacttgaactacatattactttctatttagaagatagttttgatgaggatacagtagcttaactgttagtaatacacgaacagaaaatcttttattgctaaaatccagctctttagggtgcaacatggcatattctttatatagcaccatgatgctctctttgaaactgagcttgcaatatgggatacttcattgacaacatcaattaataaaatgtaagtcaaatttttgtgcctggatggtacaaatgtaatcaccaaagaaatctgtcacataaaaacactggtggcatttctcaagtgatgcccattactcttgactttactatgtcaatggaacacacagctaagggcttctacatcttggaatggcagtctcagacttgccccacctcttaaattagacatgaaatagaaacatagaatagatgctactctaaagtcacaatggaaatgcccaacacatttcacaaatacaattatatgtaaacaaaaagagaactctatgtatcaaaatgactttgcaagtttaaatacaatattgatgcatctatggcaattttcacatagcccttgaaaagcaccaggtagcttggtgttattatatgactttatcccctagaaaagaatgaacaggtctgaaaagaccttctagattattcacatgagaaaaagggtaagaaaataatagtaaccaataatataacctgtgatgttggagaaacctggaagggcatttatagtctaatatgatattaattactaagttaaacattttattaggagaataaaaaaattcagaaaaaaacaatatggcgcaattttaagtgaaaagaagtatagatgataatagctaccttcaagagaacatgtaaaagtaaattcaataactcctggggcaggttcaaaagaggtaatgctgcatcaaaatggctatgtaaagaataatgggggcatattaccataatcgatatcaagaaaatggatatatgtatatagcagaaaaaatctggggctcatttaaaattaattctagttttaaaaaaatcattaacaaaaacgtatattgtcattaaagagaaatttccattgaaggagaagttgaaaaaattctgtagaggttctattgtatcttagtctaactcctatcttgattctgtgcaatgaagctatgttattaggtaaaatagtattataaatcaagctctttgggaaatttgctggcctaggtacatgacagagccacattttataatacaattatgtaaatcataacaaagtcccagagtttaagtgctcatccttctacgtggaatgaaattactacaaaatggtatcacagcattatggaaatatttcagatcacgttataatcaagtcagaataaacggggattgaaaccacagacattatgttaacataagaatgctatttataaattcaattgtatcataaaggcatggctaagctaaagctaaagtgagaactaacaagttcaccagtaaaagttacctgaattttataacagatgaatgatatcatactcatcatttttttaaaacacaaagctaaccaaataataaaaatcctttttccagtagataggagtagtgccttcttcactctttataacctgttcctggggtaatttccaaccttttccaagccctggcacatgtagaaagtgctaatattcatgtagcacatttgggacaatggcaaccaacatctctccctgcccatttgtacctccatgcataccgtgtactgctgccctgattttgagaatatggtatcattcacctaaagaacaccaagtgtggaaaaagctctttctaccccctaacatcctctaaatagtgatataactcttggggaaatgtatgaataaataaatccattgcaagtttaaatgaattttaaatggtgtttaccaaaaggtgttttttttcgttatggtgcacaacagcaggcatggtgataaatctcattcaagaaacagatttaggaggggacaaaaatgctaagattcttttactccataatttaaaaagcctgttctaactcatacacttttaattaggcaataaataccaagcaaaagaaacttaaaaatcatgactcatttcaaaacttcattacagacataagaagaggtaggggagcagaaatacagccttttgtgtttataaatacctcaaagcctcaaataaccaactggaaaatatacatacagagtaagaaaaggaaagcctttgacttcactgttatgttgagattattttgtaaagacaaaaagcaaaaaaattttaaaaaaataaaaaggaaatagtatatgtataatttaaaaaagaaagttatacaaaccataaaagagtaccataaacacactcctactgagcacattttagaaagattatgaaacaaaattttttgttcattagatgaagtctcttcaaaggtgctttctcttcctttgtgagtgaaaaagcccttaccccaaagccacaaagtgaaatctaccaccaaagagtgctaataaatagcagacttcctgcttcagttggtaaaaccagctgctgatttattaggtatctagagcggcaggttcatcctgttccagataggatactcatctgcagcaaaggctacttagagagatttcacacctgctgatgtgggttggactacatcttcctataactcgttccagcattcttccaacagatgcacacgctgcttctccttccgggaaacagcacatggagtccaagcacttgatacctgcatttgtttcagtaagctagtgcacgcaacaactgtcctgctggctgcaagcctcagctagcaggtgcctactgtcctcccctctgtgctggctttcagcaaattcatatgctgagctgactgaacccttatcttcttccatctaagtttgctcagctgattccttgccctcgacaatggctgcagtgcgatgaactcgtcacttaaagcaactgtgttggagtacatctgtgccttttcagtacttgtagggtggaggtgtcggtcaaagaccttctttatgatatcaagaaatagacatgtaacaaccatgaggattatggcaaaccaagcagaaccacttgacaggagctgaataaacacaaaatacatattctgggagcccaaaaatggccagagaatccctccataaaacaaggaaaatacaaaataaaatataatagatccccaggtaacgagatggttgatccaagtccaaaaatgagtttccagagccatctttactgtgactgtaataaccatgactgtgaagaccaaagtgccaaatgtccagtttccaaacatctggccatttccaagcagagatgtatctttccctattagtaaataggatccaaaaaagaaaataaaggcatgactgaagcccaggatggtccaataaagaaatgttttaatacttaagaggcggtttttactaatgtctcgataaagggtgggcttattttgtaacacatgagggtctacatgctgttccaaaagactatatatcagaataggtagggaagtaaaacaaatattgtataaagtcaggtacacgctgtcatacaatgtttgctgagaaaacaaacagtagaactgatataaaaactggggtgtgataaagcacacattcttataaaaaaaatactgtacaagggtagctattctaatataataaaaatgaccatgaacaaaaagcaatttggagaggaacttaaatctggctattgcatagtcactgtttcttgcagcctgtcttccttctttacccatgattcctatgccaacatgggcttcttgtatcatgcttacgtcattagcaccatcaccaacagccaatgttataggtttctcaggtgatatttttattagtcttattacttttgctttctgcagtggagccatacgacagcataatacagctgaacaatttctgcaaacttccataaatagtttttcatgctccctgagtgcaagagataggctggtcccatccactaccagcccatgctgaatcacatgatcctctgtaattcttctggcaagctgcctcaattgttcagcacactcgctgtctgatttctggtttataagttcaaggatgttcatggttctatgaaaatggccacatgataaactcacactaacagctgtttcatgtttatccccagtaagtacccatactttgataccagccattctcaatgcttcaatagtttctcgaactttatcttgtagtctgtcttctactgctgtggctccaagtaatatcaggtctttctctatgaactggaaaacagctgccaatttctcttcccgctgctgcaaggcagtcctggcttcaaatatgcgtttatctatttcctcatactcttttgatgtaaattttctatatgctatacacagagttcttagccctttcaaagcaaattcatctacatgaattctggttttttctatttctccacctatacatttagggagaattgatgactcagctcctttagcaaataataacttctcacctgaaggtgcctgaacaattacactcattctcctacgatctgaatcaaattccagaatatgaagcagtttgtaccgttccagttttccaagagttttaacctccatagtttcttcagaattgccaataaacacaataccaatccttgcagcagcttctactagagccttttcatctggtgaagatgcatagtactccaactgcgatggtgccaggttggattgccagggaccatcaccagtgcagtcagtttgaacattgctaatctgtacagtgtgacagagactgactgctttaaagaagagatcatgttctttaattagttcagtttcattttcaggactggttctgaaagaggaactggttgtaagatgggataagttgttaagatgggataaactactaagataagataagtttccttctgaagagtctggtgttggtccttcgggtacaagtctaccattaatttcttggtatttcatgccattaattgaacattcccgaaactgcatctcattttctgtcagtgtaccagttttatctgtaaacacgtactctacctgtccaagctcttcattcagatcggaagtattgacttgagctttctgatctgattcttcatgatacagatcaagatcccagccaataaaaaatgatccaagaaatttctgcatttcgactgtcacatataatgaaattggaatgatgaaattgtagagaaccaaaaaagcaaggaagtctgaaataaatctcagaatcttactgctatttctttgatgttctgttttttggttataccaaggttcatcccatttttcttcagcttgccatgtatacttcaagatagtgctgatgacagcttcagatataagaattactagataaattatcaaaaatgtattcattgacttttctactgcagatcgtttctgtgatttgctcttgtaatttaatgccatcttagtttccattccagtgtataccgcaacaccaaaaatttcttttgtgttttttaatctggctccacgaagcaggagactctccggccccagaggtcttacaatttcttccatttgttgggttatgatcattcgtcccatgaatctgtataagtctgcttctggttgctggcattctattacagctactagagtgtccaaattggcaactgtttgtaataatgctgtttctggaactgccacatgtgtcttcaggttagtttctccgtccaaactagcagttgtaacgtgacaggaaccatccagtcgatctgaggacagaagcaccaagtctgcaggaaaaatttcatctttggctattcgaacaatatcacccacccgaatgttttttgatctagtttttacaaggccaccacttcgaacaacataaacaggagctccatttacttcattatctgagttatgccgtaaccaatcttcatatccctgctttatggcagttactgttatcacaaagaataatggaagtccactggtaactggactggtaggtgtatcaatcataagctgaaccaaaaatataataagaaaataaaagtttgccactcttctgaactgttcaaataaattttttggaacaaaattccacacagtgtacttagatgaaatgatcctgttatctataaatttctgaggtgtgtaaaggccattctgaggaaacctgttggctacgtagatggttcttgtgtcactctgatgtggtgggtcaaaacccagctgctgccggatccagcgccacattcccccgtcgtcgccgtccgggtcccgcggggcgcgggggccgcggggctgcaggtggaggccgacaagacagaggcgggagcgggcgagcccctcgggccgaagttccgcttaccgccgccgccgccactgcctcactccccgcgccgcgtccccatcccgcggcgtcggccccgagtcctacaggcgcggccccggcgccgcccccgcccggcgcagctgagcctgccgccgcgccgcagccaccttcattatt

SEQ ID NO: 8957 - RNA, 6963 nt, Homo sapiens
  source 1..6963: mol_type = other RNA
accctttttctctttcccagagatgctaagtttgtatgtagctcaactttaattcgactagtttctagaaaagctggaacagtatctaccttaggttagggaaggacttgttcactactgtctccctagcatctagaactgtgtctgacatatattgggcacccagtatttgcagaataaatgaataaaatgagaagatgaaaatttcttaaagagtaagtatttacaggggacaagtatgcttttaactataacttttaactataacagctatcagtactccaattatccggagtcagatgtccaattccaaactgccaatactttatattagtttttcttctttccacattgcttacacagaataatcttattaggtaaagtctccttcattttaaattttttttcaaagcacacatgtgcattcatatgttaaatataatttttgacagaacattaaacacttgaactacatattactttctatttagaagatagttttgatgaggatacagtagcttaactgttagtaatacacgaacagaaaatcttttattgctaaaatccagctctttagggtgcaacatggcatattctttatatagcaccatgatgctctctttgaaactgagcttgcaatatgggatacttcattgacaacatcaattaataaaatgtaagtcaaatttttgtgcctggatggtacaaatgtaatcaccaaagaaatctgtcacataaaaacactggtggcatttctcaagtgatgcccattactcttgactttactatgtcaatggaacacacagctaagggcttctacatcttggaatggcagtctcagacttgccccacctcttaaattagacatgaaatagaaacatagaatagatgctactctaaagtcacaatggaaatgcccaacacatttcacaaatacaattatatgtaaacaaaaagagaactctatgtatcaaaatgactttgcaagtttaaatacaatattgatgcatctatggcaattttcacatagcccttgaaaagcaccaggtagcttggtgttattatatgactttatcccctagaaaagaatgaacaggtctgaaaagaccttctagattattcacatgagaaaaagggtaagaaaataatagtaaccaataatataacctgtgatgttggagaaacctggaagggcatttatagtctaatatgatattaattactaagttaaacattttattaggagaataaaaaaattcagaaaaaaacaatatggcgcaattttaagtgaaaagaagtatagatgataatagctaccttcaagagaacatgtaaaagtaaattcaataactcctggggcaggttcaaaagaggtaatgctgcatcaaaatggctatgtaaagaataatgggggcatattaccataatcgatatcaagaaaatggatatatgtatatagcagaaaaaatctggggctcatttaaaattaattctagttttaaaaaaatcattaacaaaaacgtatattgtcattaaagagaaatttccattgaaggagaagttgaaaaaattctgtagaggttctattgtatcttagtctaactcctatcttgattctgtgcaatgaagctatgttattaggtaaaatagtattataaatcaagctctttgggaaatttgctggcctaggtacatgacagagccacattttataatacaattatgtaaatcataacaaagtcccagagtttaagtgctcatccttctacgtggaatgaaattactacaaaatggtatcacagcattatggaaatatttcagatcacgttataatcaagtcagaataaacggggattgaaaccacagacattatgttaacataagaatgctatttataaattcaattgtatcataaaggcatggctaagctaaagctaaagtgagaactaacaagttcaccagtaaaagttacctgaattttataacagatgaatgatatcatactcatcatttttttaaaacacaaagctaaccaaataataaaaatcctttttccagtagataggagtagtgccttcttcactctttataacctgttcctggggtaatttccaaccttttccaagccctggcacatgtagaaagtgctaatattcatgtagcacatttgggacaatggcaaccaacatctctccctgcccatttgtacctccatgcataccgtgtactgctgccctgattttgagaatatggtatcattcacctaaagaacaccaagtgtggaaaaagctctttctaccccctaacatcctctaaatagtgatataactcttggggaaatgtatgaataaataaatccattgcaagtttaaatgaattttaaatggtgtttaccaaaaggtgttttttttcgttatggtgcacaacagcaggcatggtgataaatctcattcaagaaacagatttaggaggggacaaaaatgctaagattcttttactccataatttaaaaagcctgttctaactcatacacttttaattaggcaataaataccaagcaaaagaaacttaaaaatcatgactcatttcaaaacttcattacagacataagaagaggtaggggagcagaaatacagccttttgtgtttataaatacctcaaagcctcaaataaccaactggaaaatatacatacagagtaagaaaaggaaagcctttgacttcactgttatgttgagattattttgtaaagacaaaaagcaaaaaaattttaaaaaaataaaaaggaaatagtatatgtataatttaaaaaagaaagttatacaaaccataaaagagtaccataaacacactcctactgagcacattttagaaagattatgaaacaaaattttttgttcattagatgaagtctcttcaaaggtgctttctcttcctttgtgagtgaaaaagcccttaccccaaagccacaaagtgaaatctaccaccaaagagtgctaataaatagcagacttcctgcttcagttggtaaaaccagctgctgatttattaggtatctagagcggcaggttcatcctgttccagataggatactcatctgcagcaaaggctacttagagagatttcacacctgctgatgtgggttggactacatcttcctataactcgttccagcattcttccaacagatgcacacgctgcttctccttccgggaaacagcacatggagtccaagcacttgatacctgcatttgtttcagtaagctagtgcacgcaacaactgtcctgctggctgcaagcctcagctagcaggtgcctactgtcctcccctctgtgctggctttcagcaaattcatatgctgagctgactgaacccttatcttcttccatctgtgccttttcagtacttgtagggtggaggtgtcggtcaaagaccttctttatgatatcaagaaatagacatgtaacaaccatgaggattatggcaaaccaagcagaaccacttgacaggagctgaataaacacaaaatacatattctgggagcccaaaaatggccagagaatccctccataaaacaaggaaaatacaaaataaaatataatagatccccaggtaacgagatggttgatccaagtccaaaaatgagtttccagagccatctttactgtgactgtaataaccatgactgtgaagaccaaagtgccaaatgtccagtttccaaacatctggccatttccaagcagagatgtatctttccctattagtaaataggatccaaaaaagaaaataaaggcatgactgaagcccaggatggtccaataaagaaatgttttaatacttaagaggcggtttttactaatgtctcgataaagggtgggcttattttgtaacacatgagggtctacatgctgttccaaaagactatatatcagaataggtagggaagtaaaacaaatattgtataaagtcaggtacacgctgtcatacaatgtttgctgagaaaacaaacagtagaactgatataaaaactggggtgtgataaagcacacattcttataaaaaaaatactgtacaagggtagctattctaatataataaaaatgaccatgaacaaaaagcaatttggagaggaacttaaatctggctattgcatagtcactgtttcttgcagcctgtcttccttctttacccatgattcctatgccaacatgggcttcttgtatcatgcttacgtcattagcaccatcaccaacagccaatgttataggtttctcaggtgatatttttattagtcttattacttttgctttctgcagtggagccatacgacagcataatacagctgaacaatttctgcaaacttccataaatagtttttcatgctccctgagtgcaagagataggctggtcccatccactaccagcccatgctgaatcacatgatcctctgtaattcttctggcaagctgcctcaattgttcagcacactcgctgtctgatttctggtttataagttcaaggatgttcatggttctatgaaaatggccacatgataaactcacactaacagctgtttcatgtttatccccagtaagtacccatactttgataccagccattctcaatgcttcaatagtttctcgaactttatcttgtagtctgtcttctactgctgtggctccaagtaatatcaggtctttctctatgaactggaaaacagctgccaatttctcttcccgctgctgcaaggcagtcctggcttcaaatatgcgtttatctatttcctcatactcttttgatgtaaattttctatatgctatacacagagttcttagccctttcaaagcaaattcatctacatgaattctggttttttctatttctccacctatacatttagggagaattgatgactcagctcctttagcaaataataacttctcacctgaaggtgcctgaacaattacactcattctcctacgatctgaatcaaattccagaatatgaagcagtttgtaccgttccagttttccaagagttttaacctccatagtttcttcagaattgccaataaacacaataccaatccttgcagcagcttctactagagccttttcatctggtgaagatgcatagtactccaactgcgatggtgccaggttggattgccagggaccatcaccagtgcagtcagtttgaacattgctaatctgtacagtgtgacagagactgactgctttaaagaagagatcatgttctttaattagttcagtttcattttcaggactggttctgaaagaggaactggttgtaagatgggataagttgttaagatgggataaactactaagataagataagtttccttctgaagagtctggtgttggtccttcgggtacaagtctaccattaatttcttggtatttcatgccattaattgaacattcccgaaactgcatctcattttctgtcagtgtaccagttttatctgtaaacacgtactctacctgtccaagctcttcattcagatcggaagtattgacttgagctttctgatctgattcttcatgatacagatcaagatcccagccaataaaaaatgatccaagaaatttctgcatttcgactgtcacatataatgaaattggaatgatgaaattgtagagaaccaaaaaagcaaggaagtctgaaataaatctcagaatcttactgctatttctttgatgttctgttttttggttataccaaggttcatcccatttttcttcagcttgccatgtatacttcaagatagtgctgatgacagcttcagatataagaattactagataaattatcaaaaatgtattcattgacttttctactgcagatcgtttctgtgatttgctcttgtaatttaatgccatcttagtttccattccagtgtataccgcaacaccaaaaatttcttttgtgttttttaatctggctccacgaagcaggagactctccggccccagaggtcttacaatttcttccatttgttgggttatgatcattcgtcccatgaatctgtataagtctgcttctggttgctggcattctattacagctactagagtgtccaaattggcaactgtttgtaataatgctgtttctggaactgccacatgtgtcttcaggttagtttctccgtccaaactagcagttgtaacgtgacaggaaccatccagtcgatctgaggacagaagcaccaagtctgcaggaaaaatttcatctttggctattcgaacaatatcacccacccgaatgttttttgatctagtttttacaaggccaccacttcgaacaacataaacaggagctccatttacttcattatctgagttatgccgtaaccaatcttcatatccctgctttatggcagttactgttatcacaaagaataatggaagtccactggtaactggactggtaggtgtatcaatcataagctgaaccaaaaatataataagaaaataaaagtttgccactcttctgaactgttcaaataaattttttggaacaaaattccacacagtgtacttagatgaaatgatcctgttatctataaatttctgaggtgtgtaaaggccattctgaggaaacctgttggctacgtagatggttcttgtgtcactctgatgtggtgggtcaaaacccagctgctgccggatccagcgccacattcccccgtcgtcgccgtccgggtcccgcggggcgcgggggccgcggggctgcaggtggaggccgacaagacagaggcgggagcgggcgagcccctcgggccgaagttccgcttaccgccgccgccgccactgcctcactccccgcgccgcgtccccatcccgcggcgtcggccccgagtcctacaggcgcggccccggcgccgcccccgcccggcgcagctgagcctgccgccgcgccgcagccaccttcattatt

SEQ ID NO: 8958 - RNA, 6733 nt, Homo sapiens
  source 1..6733: mol_type = other RNA
accctttttctctttcccagagatgctaagtttgtatgtagctcaactttaattcgactagtttctagaaaagctggaacagtatctaccttaggttagggaaggacttgttcactactgtctccctagcatctagaactgtgtctgacatatattgggcacccagtatttgcagaataaatgaataaaatgagaagatgaaaatttcttaaagagtaagtatttacaggggacaagtatgcttttaactataacttttaactataacagctatcagtactccaattatccggagtcagatgtccaattccaaactgccaatactttatattagtttttcttctttccacattgcttacacagaataatcttattaggtaaagtctccttcattttaaattttttttcaaagcacacatgtgcattcatatgttaaatataatttttgacagaacattaaacacttgaactacatattactttctatttagaagatagttttgatgaggatacagtagcttaactgttagtaatacacgaacagaaaatcttttattgctaaaatccagctctttagggtgcaacatggcatattctttatatagcaccatgatgctctctttgaaactgagcttgcaatatgggatacttcattgacaacatcaattaataaaatgtaagtcaaatttttgtgcctggatggtacaaatgtaatcaccaaagaaatctgtcacataaaaacactggtggcatttctcaagtgatgcccattactcttgactttactatgtcaatggaacacacagctaagggcttctacatcttggaatggcagtctcagacttgccccacctcttaaattagacatgaaatagaaacatagaatagatgctactctaaagtcacaatggaaatgcccaacacatttcacaaatacaattatatgtaaacaaaaagagaactctatgtatcaaaatgactttgcaagtttaaatacaatattgatgcatctatggcaattttcacatagcccttgaaaagcaccaggtagcttggtgttattatatgactttatcccctagaaaagaatgaacaggtctgaaaagaccttctagattattcacatgagaaaaagggtaagaaaataatagtaaccaataatataacctgtgatgttggagaaacctggaagggcatttatagtctaatatgatattaattactaagttaaacattttattaggagaataaaaaaattcagaaaaaaacaatatggcgcaattttaagtgaaaagaagtatagatgataatagctaccttcaagagaacatgtaaaagtaaattcaataactcctggggcaggttcaaaagaggtaatgctgcatcaaaatggctatgtaaagaataatgggggcatattaccataatcgatatcaagaaaatggatatatgtatatagcagaaaaaatctggggctcatttaaaattaattctagttttaaaaaaatcattaacaaaaacgtatattgtcattaaagagaaatttccattgaaggagaagttgaaaaaattctgtagaggttctattgtatcttagtctaactcctatcttgattctgtgcaatgaagctatgttattaggtaaaatagtattataaatcaagctctttgggaaatttgctggcctaggtacatgacagagccacattttataatacaattatgtaaatcataacaaagtcccagagtttaagtgctcatccttctacgtggaatgaaattactacaaaatggtatcacagcattatggaaatatttcagatcacgttataatcaagtcagaataaacggggattgaaaccacagacattatgttaacataagaatgctatttataaattcaattgtatcataaaggcatggctaagctaaagctaaagtgagaactaacaagttcaccagtaaaagttacctgaattttataacagatgaatgatatcatactcatcatttttttaaaacacaaagctaaccaaataataaaaatcctttttccagtagataggagtagtgccttcttcactctttataacctgttcctggggtaatttccaaccttttccaagccctggcacatgtagaaagtgctaatattcatgtagcacatttgggacaatggcaaccaacatctctccctgcccatttgtacctccatgcataccgtgtactgctgccctgattttgagaatatggtatcattcacctaaagaacaccaagtgtggaaaaagctctttctaccccctaacatcctctaaatagtgatataactcttggggaaatgtatgaataaataaatccattgcaagtttaaatgaattttaaatggtgtttaccaaaaggtgttttttttcgttatggtgcacaacagcaggcatggtgataaatctcattcaagaaacagatttaggaggggacaaaaatgctaagattcttttactccataatttaaaaagcctgttctaactcatacacttttaattaggcaataaataccaagcaaaagaaacttaaaaatcatgactcatttcaaaacttcattacagacataagaagaggtaggggagcagaaatacagccttttgtgtttataaatacctcaaagcctcaaataaccaactggaaaatatacatacagagtaagaaaaggaaagcctttgacttcactgttatgttgagattattttgtaaagacaaaaagcaaaaaaattttaaaaaaataaaaaggaaatagtatatgtataatttaaaaaagaaagttatacaaaccataaaagagtaccataaacacactcctactgagcacattttagaaagattatgaaacaaaattttttgttcattagatgaagtctcttcaaaggtgctttctcttcctttgtgagtgaaaaagcccttaccccaaagccacaaagtgaaatctaccaccaaagagtgctaataaatagcagacttcctgcttcagttggtaaaaccagctgctgatttattaggtatctagagcggcaggttcatcctgttccagataggatactcatctgcagcaaaggctacttagagagatttcacacctgctgatgtgggttggactacatcttcctataactcgttccagcattcttccaacagatgcacacgctgcttctccttccgggaaacagcacatggagtccaagcacttgatacctgcatttgtttcagtaagctagtgcacgcaacaactgtcctgctggctgcaagcctcagctagcaggtgcctactgtcctcccctctgtgctggctttcagcaaattcatatgctgagctgactgaacccttatcttcttccatctgtgccttttcagtacttgtagggtggaggtgtcggtcaaagaccttctttatgatatcaagaaatagacatgtaacaaccatgaggattatggcaaaccaagcagaaccacttgacaggagctgaataaacacaaaatacatattctgggagcccaaaaatggccagagaatccctccataaaacaaggaaaatacaaaataaaatataatagatccccaggtaacgagatggttgatccaagtccaaaaatgagtttccagagccatctttactgtgactgtaataaccatgactgtgaagaccaaagtgccaaatgtccagtttccaaacatctggccatttccaagcagagatgtatctttccctattagtaaataggatccaaaaaagaaaataaaggcatgactgaagcccaggatggtccaataaagaaatgttttaatacttaagaggcggtttttactaatgtctcgataaagggtgggcttattttgtaacacatgagggtctacatgctgttccaaaagactatatatcagaataggtagggaagtaaaacaaatattgtataaagtcaggtacacgctgtcatacaatgtttgctgagaaaacaaacagtagaactgatataaaaactggggtgtgataaagcacacattcttataaaaaaaatactgtacaagggtagctattctaatataataaaaatgaccatgaacaaaaagcaatttggagaggaacttaaatctggctattgcatagtcactgtttcttgcagcctgtcttccttctttacccatgattcctatgccaacatgggcttcttgtatcatgcttacgtcattagcaccatcaccaacagccaatgttataggtttctcaggtgatatttttattagtcttattacttttgctttctgcagtggagccatacgacagcataatacagctgaacaatttctgcaaacttccataaatagtttttcatgctccctgagtgcaagagataggctggtcccatccactaccagcccatgctgaatcacatgatcctctgtaattcttctggcaagctgcctcaattgttcagcacactcgctgtctgatttctggtttataagttcaaggatgttcatggttctatgaaaatggccacatgataaactcacactaacagctgtttcatgtttatccccagtaagtacccatactttgataccagccattctcaatgcttcaatagtttctcgaactttatcttgtagtctgtcttctactgctgtggctccaagtaatatcaggtctttctctatgaactggaaaacagctgccaatttctcttcccgctgctgcaaggcagtcctggcttcaaatatgcgtttatctatttcctcatactcttttgatgtaaattttctatatgctatacacagagttcttagccctttcaaagcaaattcatctacatgaattctggttttttctatttctccacctatacatttagggagaattgatgactcagctcctttagcaaataataacttctcacctgaaggtgcctgaacaattacactcattctcctacgatctgaatcaaattccagaatatgaagcagtttgtaccgttccagttttccaagagttttaacctccatagtttcttcagaattgccaataaacacaataccaatccttgcagcagcttctactagagccttttcatctggtgaagatgcatagtactccaactgcgatggtgccaggttggattgccagggaccatcaccagtgcagtcagtttgaacattgctaatctgtacagtgtgacagagactgactgctttaaagaagagatcatgttctttaattagttcagtttcattttcaggactggttctgaaagaggaactggttgtaagatgggataagttgttaagatgggataaactactaagataagataagtttccttctgaagagtctggtgttggtccttcgggtacaagtctaccattaatttcttggtatttcatgccattaattgaacattcccgaaactgcatctcattttctgtcagtgtaccagttttatctgtaaacacgtactctacctgtccaagctcttcattcagatcggaagtattgacttgagctttctgatctgattcttcatgatacagatcaagatcccagccaataaaaaatgatccaagaaatttctgcatttcgactgtcacatataatgaaattggaatgatgaaattgtagagaaccaaaaaagcaaggaagtctgaaataaatctcagaattgctatttctttgatgttctgttttttggttataccaaggttcatcccatttttcttcagcttgccatgtatacttcaagatagtgctgatgacagcttcagatataagaattactagataaattatcaaaaatgtattcattgacttttctactgcagatcgtttctgtgatttgctcttgtaatttaatgccatcttagtttccattccagtgtataccgcaacaccaaaaatttcttttgtgttttttaatctggctccacgaagcaggagactctccggccccagaggtattgcatacttcttgaagcacaggtcttcttgctgtttgaatttctctccataaaggagatataaaacgacaaggaataacttacaatttcttccatttgttgggttatgatcattcgtcccatgaatctgtataagtctgcttctggttgctggcattctattacagctactagagtgtccaaattggcaactgtttgtaataatgctgtttctggaactgccacatgtgtcttcaggttagtttctccgtccaaactagcagttgtaacgtgacaggaaccatccagtcgatctgaggacagaagcaccaagtctgcaggaaaaatttcatctttggctattcgaacaatatcacccacccgaatgttttttgatctagtttttacaaggccaccacttcgaacaacataaacaggagctccatttacttcattatctgagttatgccgtaaccaatcttcatatccctgctttatggcagttactgttatcacaaagaataatggaagtccactggtaactggactggtaggtgtatcaatcataagctgaaccaaaaatataataagaaaataaaagtttgccactcttctgaactgttcaaataaattttttggaacaaaattccacacagtgtacttagatgaaatgatcctgttatctataaatttctgaggtgtgtaaaggccattctgaggaaacctgttggctacgtagatggttcttgtgtcac

SEQ ID NO: 8959 - RNA, 3168 nt, Homo sapiens
  source 1..3168: mol_type = other RNA
accctttttctctttcccagaggtggcggctgacagagcccagaccctgatccccagtcccttgtggtctcttgtctgctaggctggcccctaggaagtcttggatgaacagaggcagtgggttgaggggagaataccctcagcgggcatctctccagcggccagtttgtgtacagctgtcataagtttctctgggccacccccaacccatgcctgcatccctctcaccttagcatccactgtcatatcacatgaagccgcaccacagtgcagtgctgtgactgtcggcctcctactggctctgaatagtctcggccccactagagttcagccaccacgtcctccccctgatgttgctgcagtgctacctctttggggatggaggtgtgatctgtgggtgaactggcaaatcctgtccccacgtgcaaatgaaatcacagccaaagggcctcccttgtccctgactagcaagcacgggactttttctctgctgtggatctgcagaggacatatgccctttagctgtggaagggattcacagaaggccagggctgcaacctgtgacctcagacctccgctggctgcgagacggcggctgggcccgaggcgggagtgggctcggtttccttcgctggcgcaccttctgatgatgccccggcaacagacctggcctgggggtgcaggctggccctggatcgccggacggtcttctcgccggtatggatcctctggtggtggaagagggccgggcgctcacggaaggcgcggccacactgcgtacacacgaagggcttctcgcccgtgtgaatgcgccggtggctgagcagcacggcgcccttggcgaaggccttgccacagtccacgcagcggaagggccgctcgcccgtgtgcaggagctggtgctgggtgaggttggagctgtggctaaaggcgcggccgcactgtgggcaggcgaagggcttctcgcctgtgtgcacgcgctggtgcttaaagagcgaggagccctggctgaaggcagcaccgcagagcgcgcacacgaagggcttctcgcctgtgtgcgtacgctcgtgctggatcaggtgcgagttgcggcagaagcggcggccacactgtgcgcaagcataaggacgcccacccgcgtggatcttgcggtgctggctgaggttggagccgtggctgaaggccttgccgcactcggagcagcggaaggacttctcggccgtgtggatgcgctggtgccgcaccagcgaggagctatgccggaaggccttgccgcacacggggcacgcgtagggcgtctcgccgctgtggatgcgctggtgctgcgtcaagtgcgacgtctggctgaaggccttgccgcactgggcgcactcgtagggccgctccccggtgtgggtgcgtaggtgcttgaggaggtcggagctcttcacgaacactttgctgcacgccctgcattcgaaggacttctccccagcgtgaagagcctcgcccagctcgtcccaggtcgagggctcctggccaccgaggagtctatgaggctcctgccaaactgcacccattcggtgatgtccccgaccgccggcagcctccaggtcctgggcgctcccaaaggttctcccagggacctcctgtgcacatggtttctgccgctcaggcgtcctgggctgcctccccagcaacgcatgctctgtgagtgtcttttctctaagccggacgccctcgggaggcctaagcggggaggtcagtcgcaggctgacgctggcttgcccactgcctgagcctagcaggagcctctcccagtagatcaccgacacccccgtgggttttctctcccgagatggggaggcaccccgttgtctctgcaggctttttacactgtggcaggcaccggcaacagggaagacgctagtagtcatcccaggtggggtatctgggaaagctcgtggccattctccagaaacatctctatcctctgtcaaactccaggaaccagggttgcgcctcctgtaggtggtcctggacagggttgtgtccgttccactgggaacccagggctcctcgccacgctccagttggatgaccacacgaggtcgagaggtggagagtcccagcgaggccacaagtgcgaagttgtctagcatcacgcggcggtacagggccctctgggctgtgtccaggagcccccactcctcctgggagaagtacacagccacatcctcaaaggccatctggtcctgggacatcccagactcttgatctttcccctgaaggaaacctgctttcctttcaattctcctttctatctacagcagctctcttcttccaggcgctcaggctgaacaacatggggtacttagttcttcaaacagcccacacctgatgcatccgcagatccaccagaattcacctggtcgcccacctccactgctgcccagactgtggcagtcggttcttcccttcatgccgacacccctgcatgtctgttctccacgcaacaaacggtggaaccgttttaaagtcctcagaggatgtcctgattctgttcaaaacttctatgtctcccgacgccctcgagataaagcccactccctcgcctgatactgcagccgcacacatcccctctactccagctccacatcgagagagctcagtcccagaagcacctgggcttcggctcccctcccaggttttgcacacgcaggactctcccctcggagcctccttcgggacctcagccccctggctgcccgaactcgggagctcaccagtgccctggacgcaggagtttgcactgacccccgcaacccccccagggcagggagaggaaagacgactaggcgaggtctaggaagcggcctccctccgtgagggcgcggtctgtgtgagcagggactcccctgcttccccgacgcgggcttgtcagcgccaccgccgccagcggaacccgcagctgggagggaagaaaggcgtggaccacccagcctttccccgccagcagcgtcccggggccgccccgcgcctcagtctccccggccatcatggacgtggaacgcccagcgcgcagcctcctgggctgccgcacggtgggagagcgcatggctcccgccgcggcccgacagtcccctggacgcccacgacgcactctgagaaacagaggcttgggggcgc

SEQ ID NO: 8960 - RNA, 2338 nt, Homo sapiens
  source 1..2338: mol_type = other RNA
accctttttctctttcccagaggtggcggctgacagagcccagaccctgatccccagtcccttgtggtctcttgtctgctaggctggcccctaggaagtcttggatgaacagaggcagtgggttgaggggagaataccctcagcgggcatctctccagcggccagtttgtgtacagctgtcataagtttctctgggccacccccaacccatgcctgcatccctctcaccttagcatccactgtcatatcacatgaagccgcaccacagtgcagtgctgtgactgtcggcctcctactggctctgaatagtctcggccccactagagttcagccaccacgtcctccccctgatgttgctgcagtgctacctctttggggatggaggtgtgatctgtgggtgaactggcaaatcctgtccccacgtgcaaatgaaatcacagccaaagggcctcccttgtccctgactagcaagcacgggactttttctctgctgtggatctgcagaggacatatgccctttagctgtggaagggattcacagaaggccagggctgcaacctgtgacctcagacctccgctggctgcgagacggcggctgggcccgaggcgggagtgggctcggtttccttcgctggcgcaccttctgatgatgccccggcaacagacctggcctgggggtgcaggctggccctggatcgccggacggtcttctcgccggtatggatcctctggtggtggaagagggccgggcgctcacggaaggcgcggccacactgcgtacacacgaagggcttctcgcccgtgtgaatgcgccggtggctgagcagcacggcgcccttggcgaaggccttgccacagtccacgcagcggaagggccgctcgcccgtgtgcaggagctggtgctgggtgaggttggagctgtggctaaaggcgcggccgcactgtgggcaggcgaagggcttctcgcctgtgtgcacgcgctggtgcttaaagagcgaggagccctggctgaaggcagcaccgcagagcgcgcacacgaagggcttctcgcctgtgtgcgtacgctcgtgctggatcaggtgcgagttgcggcagaagcggcggccacactgtgcgcaagcataaggacgcccacccgcgtggatcttgcggtgctggctgaggttggagccgtggctgaaggccttgccgcactcggagcagcggaaggacttctcggccgtgtggatgcgctggtgccgcaccagcgaggagctatgccggaaggccttgccgcacacggggcacgcgtagggcgtctcgccgctgtggatgcgctggtgctgcgtcaagtgcgacgtctggctgaaggccttgccgcactgggcgcactcgtagggccgctccccggtgtgggtgcgtaggtgcttgaggaggtcggagctcttcacgaacactttgctgcacgccctgcattcgaaggacttctccccagcgtgaagagcctcgcccagctcgtcccaggtcgagggctcctggccaccgaggagtctatgaggctcctgccaaactgcacccattcggtgatgtccccgaccgccggcagcctccaggtcctgggcgctcccaaaggttctcccagggacctcctgtgcacatggtttctgccgctcaggcgtcctgggctgcctccccagcaacgcatgctctgtgagtgtcttttctctaagccggacgccctcgggaggcctaagcggggaggtcagtcgcaggctgacgctggcttgcccactgcctgagcctagcaggagcctctcccagtagatcaccgacacccccgtgggttttctctcccgagatggggaggcaccccgttgtctctgcaggctttttacactgtggcaggcaccggcaacagggaagacgctagtagtcatcccaggtggggtatctgggaaagctcgtggccattctccagaaacatctctatcctctgtcaaactccaggaaccagggttgcgcctcctgtaggtggtcctggacagggttgtgtccgttccactgggaacccagggctcctcgccacgctccagttggatgaccacacgaggtcgagaggtggagagtcccagcgaggccacaagtgcgaagttgtctagcatcacgcggcggtacagggccctctgggctgtgtccaggagcccccactcctcctgggagaagtacacagccacatcctcaaaggccatctggtccttcctcgccgccagcctcgagcaccaggaaccccctggaaaccggacccgacccgcggtccccagcccagaccaccggtgtggcctgacgcgggcggcgaagt

SEQ ID NO: 8961 - RNA, 122 nt, Homo sapiens
  source 1..122: mol_type = other RNA
accctttttctctttcccagatattggctttataaacctttgatatcaaagcctgtatgttccgattcttcttggtgtctctgtctttgagggtacttctggaatgaaggttcttatgacct

SEQ ID NO: 8962 - RNA, 184 nt, Homo sapiens
  source 1..184: mol_type = other RNA
accctttttctctttcccagatattggctttataaacctttgatatcaaagcctgtatgttccgattcttcttggtgtctctgtctttgagggtacttctggaatgaaggttcttatgacctactttatagaaacgtcagaggattcttttatggcctgcttcaggggagaagggtgggagaag

SEQ ID NO: 8963 - RNA, 197 nt, Homo sapiens
  source 1..197: mol_type = other RNA
accctttttctctttcccagatattggctttataaacctttgatatcattggggttgaccaaagcctgtatgttccgattcttcttggtgtctctgtctttgagggtacttctggaatgaaggttcttatgacctactttatagaaacgtcagaggattcttttatggcctgcttcaggggagaagggtgggagaag

SEQ ID NO: 8964 - RNA, 693 nt, Homo sapiens
  source 1..693: mol_type = other RNA
accctttttctctttcccagtagcctcctgtctggctcgctcagttgtttctccagtaatcttttctcctggaggagctgggcctgtacttcccgtgtctttgaagctgtctcagcttggactttctttgtctcctcctgtaatgtctgtatttctttctcctgcttttcctttaatatagcaatgtccctcattgcctgcaacttccgcttcaaactggattggatattttccttttgcaagagcgctgttttaagcactgaaatttgttctgcatatctggaggctgattcttgtcttcttcgttcaatctctccacttttttgtaaatagctgttccataccttctcaggttgctctgtgtactcttcagttttgttagtcaggtattccagaaagaatctgttttcagcctggacaagtaacttttctcggtgtagctccctggattcctccagtagctgtttccgctgggtttgagcttgttttatatgcttgttcagatccgtcatttccgccactatcttttctttaagccttgtctctacctttgttagcttctctggcttgacaaaattatttattagactatgatacggtggaaggagccttctggggccctcagcaaacccgctcctttctgacgctgtggtggttttcgttcgcagcccagaacattgcggaagtttctct

SEQ ID NO: 8965 - RNA, 1247 nt, Homo sapiens
  source 1..1247: mol_type = other RNA
accctttttctctttcccagtagcctcctgtctggctcgctcagttgtttctccagtaatcttttctcctggaggagctgggcctgtacttcccgtgtctttgaagctgtctcagcttggactttctttgtctcctcctgtaatgtctgtatttctttctcctgcttttcctttaatatagcaatgtccctcattgcctgcaacttccgcttcaaactggattggatattttccttttgcaagagcgctgttttaagcactgaaatttgttctgcatatctggaggctgattcttgtcttcttcgttcaatctctccacttttttgtaaatagctgttccataccttctcaggttgctctgtgtactcttcagttttgttagtcaggtattccagaaagaatctgttttcagcctggacaagtaacttttctcggtgtagctccctggattcctccagtagctgtttccgctgggtttgagcttgttttatatgcttgttcagatccgtcatttccgccactatcttttctttaagccttgtctctacctttgttagcttctctggcttgacaaaattatttattagactatgatacggtggaaggagccttctggggccctcagcaaacctggaatccaagcattcatcctgaaggtcacggcaactgtgtagttcactgagggtgactgccaaggaatgagcgctagcatcaggaacctgcgtctgcaactcgcgggaacaatgtgcaagtgtggaaagctcccgtagtttattcgttcggtgctcaaagggtctcggtgctgcccagcaaccctggagactgcaccctgctccagtcccggctggtccagccctgaactgtttaaccgcctcggctaccgaataagcccgagcagccggtcctccagtggctccgctccccgttctctgtgggctcaaaatgacaggcatgctcctcgttttcttgctgtgtgagccctgccctcgggaccccatctcttctggccttcctccgggagacaaaagccctcccaggctgcagagatcagcgcccttttcctagctcccttcagccttcctctcgcttgctcagcgcccccacttcctcgccactgtcactagttgactcatcagccctgcccgacgctaagaagatgccctggcaaccgccgcgcccctcacccgctcctttctgacgctgtggtggttttcgttcgcagcccagaacattgcggaagtttctct

SEQ ID NO: 8966 - RNA, 1230 nt, Homo sapiens
  source 1..1230: mol_type = other RNA
accctttttctctttcccagtagcctcctgtctggctcgctcagttgtttctccagtaatcttttctcctggaggagctgggcctgtacttcccgtgtctttgaagctgtctcagcttggactttctttgtctcctcctgtaatgtctgtatttctttctcctgcttttcctttaatatagcaatgtccctcattgcctgcaacttccgcttcaaactggattggatattttccttttgcaagagcgctgttttaagcactgaaatttgttctgcatatctggaggctgattcttgtcttcttcgttcaatctctccacttttttgtaaatagctgttccataccttctcaggttgctctgtgtactcttcagttttgttagtcaggtattccagaaagaatctgttttcagcctggacaagtaacttttctcggtgtagctccctggattcctccagtagctgtttccgctgggtttgagcttgttttatatgcttgttcagatccgtcatttccgccactatcttttctttaagccttgtctctacctttgttagcttctctggcttgacaaaattatttattagactatgatacggtggaaggagccttctggggccctcagcaaacttgcacctggaatccaagcattcatcctgaaggtcacggcaactgtgtagttcactgagggtgactgccaaggaatgagcgctagcatcaggaacctgcgtctgcaactcgcgggaacaatgtgcaagtgtggaaagctcccgtagtttattcgttcggtgctcaaagggtctcggtgctgcccagcaaccctggagactgcaccctgctccagtcccggctggtccagccctgaactgtttaaccgcctcggctaccgaataagcccgagcagccggtcctccagtggctccgctccccgttctctgtgggctcaaaatgacaggcatgctcctcgttttcttgctgtgtgagccctgccctcgggaccccatctcttctggccttcctccgggagacaaaagccctcccaggctgcagagatcagcgcccttttcctagctcccttcagccttcctctcgcttgctcagcgcccccacttcctcgccactgtcactagttgactcatcagccctgcccgacgctaagaagatgccctggcaaccgccgcgcccctcacccgctcctttctgacgctgtggtggttttcgttcgcagcc

SEQ ID NO: 8967 - RNA, 386 nt, Homo sapiens
  source 1..386: mol_type = other RNA
accctttttctctttcccagtccctcctagaatccatggttttgttagagaagtctatagtttcgctgctcaccacgagactgatcagctttggaactgttgcactgttttcctcttttgagcacagttcgtggaatggcctagaatgacgtgtgtgttgtgagggaagctgcaccaagccctttccctgtggcaatggactgccccattgagctagatgttgattggtagatagaaaggggcgtgccaagaatcctctcatctgattggttgcagcggaaaacctttcgctttttcttctcttcagcaagaatttcgccgcttgccgggttcctcactttaagtgtgcttcgttgcttttcgttctgttggtttcgaactttggg

SEQ ID NO: 8968 - RNA, 1381 nt, Homo sapiens
  source 1..1381: mol_type = other RNA
accctttttctctttcccagttcttccattctctcagggcacagccttctgcaattgtcttgatatttcaagtactcatcttctccccatgaagatggtgccctttcctttatcaagagatgctccagccatatggtaaaaactcaatgcagtgtccacatcattaatgttctttaggaaagtaaagaagttctccacctcctgaaatgtcagaccctttccttctttgaagtgcttcttgagctgcctctgcatggcggtcagcttcttggactgcaccccactgtaggcaagtagcatgccaccaaactgcctctcagtaattctcccatccacagggtcatggcgttcaaactcaagcttcagaacatcatgctgcagtttacgctgaaattcgaggaagtttttgattgtcagctttcccttcagatcagctccaaaaaagtaggttgtgagggctgaacacaagccagacttgagggtgttgccagtagttggacgatctctgtggcgcatacccatactggtttgggagcgaatgatgctctgaacctgttcaaattcttccatatctacttctccatctccattcaaatcaaacatcttgaaggcaatttcaaaatttctctgaggagtggaaagaacagttgtgaggaaaatgtagtctgaaaaggatatgagcccacattctccaagggtgtaaaatatactgccttcatcagcaaatttttctcgttcctgggaaattttctctgtctttccatcaaagcgttttattatatattgatccagacccaagtgttctggttgtttttcattgggtgttatggatcgcacaaaatcttctggtgtcataaacacttctgcttcaccaggctcactgatgactttcaaggtggcaaaatatcggaagattttgtctggcgtggagtaggctcgaatcctattctcatattccatcacttttctgtctctgaatccagaacgtttcttctttttctcttctgggtgaggggcaagatctgcagtctttttctcatggttacaaacatccccttcatctttattcttccctttatcaccgatgtcactttttaggttgtctacacatggtggagattctgcatgggccctcttccacaaaagaccagtacttgcagttactgcagatgctcccaggaaagccaccatcattagtcttcgccggatctggatgggctgtgatcctccatggtaccatcgagaacccacagccagttctgccaaagcagaaagtgagttcagacgaaacatcgcgtccaaacacgagctccagcagcctctcggtcaaagccgcccacctctgacagccatagagatgaaacagcggagacaaacctcc

SEQ ID NO: 8969 - RNA, 1375 nt, Homo sapiens
  source 1..1375: mol_type = other RNA
accctttttctctttcccagttcttccattctctcagggcacagccttctgcaattgtcttgatatttcaagtactcatcttctccccatgaagatggtgccctttcctttatcaagagatgctccagccatatggtaaaaactcaatgcagtgtccacatcattaatgttctttaggaaagtaaagaagttctccacctcctgaaatgtcagaccctttccttctttgaagtgcttcttgagctgcctctgcatggcggtcagcttcttggactgcaccccactgtaggcaagtagcatgccaccaaactgcctctcagtaattctcccatccacagggtcatggcgttcaaactcaagcttcagaacatcatgctgcagtttacgctgaaattcgaggaagtttttgattgtcagctttcccttcagatcagctccaaaaaagtaggttgtgagggctgaacacaagccagacttgagggtgttgccagtagttggacgatctctgtggcgcatacccatactggtttgggagcgaatgatgctctgaacctgttcaaattcttccatatctacttctccatctccattcaaatcaaacatcttgaaggcaatttcaaaatttctctgaggagtggaaagaacagttgtgaggaaaatgtagtctgaaaaggatatgagcccacattctccaagggtgtaaaatatactgccttcatcagcaaatttttctcgttcctgggaaattttctttccatcaaagcgttttattatatattgatccagacccaagtgttctggttgtttttcattgggtgttatggatcgcacaaaatcttctggtgtcataaacacttctgcttcaccaggctcactgatgactttcaaggtggcaaaatatcggaagattttgtctggcgtggagtaggctcgaatcctattctcatattccatcacttttctgtctctgaatccagaacgtttcttctttttctcttctgggtgaggggcaagatctgcagtctttttctcatggttacaaacatccccttcatctttattcttccctttatcaccgatgtcactttttaggttgtctacacatggtggagattctgcatgggccctcttccacaaaagaccagtacttgcagttactgcagatgctcccaggaaagccaccatcattagtcttcgccggatctggatgggctgtgatcctccatggtaccatcgagaacccacagccagttctgccaaagcagaaagtgagttcagacgaaacatcgcgtccaaacacgagctccagcagcctctcggtcaaagccgcccacctctgacagccatagagatgaaacagcggagacaaacctcc

SEQ ID NO: 8970 - RNA, 1543 nt, Homo sapiens
  source 1..1543: mol_type = other RNA
accctttttctctttcccagttcttccattctctcagggcacagccttctgcaattgtcttgatatttcaagtactcatcttctccccatgaagatggtgccctttcctttatcaagagatgctccagccatatggtaaaaactcaatgcagtgtccacatcattaatgttctttaggaaagtaaagaagttctccacctcctgaaatgtcagaccctttccttctttgaagtgcttcttgagctgcctctgcatggcggtcagcttcttggactgcaccccactgtaggcaagtagcatgccaccaaactgcctctcagtaattctcccatccacagggtcatggcgttcaaactcaagcttcagaacatcatgctgcagtttacgctgaaattcgaggaagtttttgattgtcagctttcccttcagatcagctccaaaaaagtaggttgtgagggctgaacacaagccagacttgagggtgttgccagtagttggacgatctctgtggcgcatacccatactggtttgggagcgaatgatgctctgaacctgttcaaattcttccatatctacttctccatctccattcaaatcaaacatcttgaaggcaatttcaaaatttctctgaggagtggaaagaacagttgtgaggaaaatgtagtctgaaaaggatatgagcccacattctccaagggtgtaaaatatactgccttcatcagcaaatttttctcgttcctgggaaattttcttttccagccactccatgattgtccttctgacttcctgttcattgtgctttgtagaaccatgcctggttctttcttctttctgaagtgctttcttcctcctctgtaaaattgaccctttacttttctttctgaccctgtgtaatattttctttttggagaatctggcctttccatcaaagcgttttattatatattgatccagacccaagtgttctggttgtttttcattgggtgttatggatcgcacaaaatcttctggtgtcataaacacttctgcttcaccaggctcactgatgactttcaaggtggcaaaatatcggaagattttgtctggcgtggagtaggctcgaatcctattctcatattccatcacttttctgtctctgaatccagaacgtttcttctttttctcttctgggtgaggggcaagatctgcagtctttttctcatggttacaaacatccccttcatctttattcttccctttatcaccgatgtcactttttaggttgtctacacatggtggagattctgcatgggccctcttccacaaaagaccagtacttgcagttactgcagatgctcccaggaaagccaccatcattagtcttcgccggatctggatgggctgtgatcctccatggtaccatcgagaacccacagccagttctgccaaagcagaaagtgagttcagacgaaacatcgcgtccaaacacgagctccagcagcctctcggtcaaagccgcccacctctgacagccatagagatgaaacagcggagacaaacctcc

SEQ ID NO: 8971 - RNA, 3348 nt, Homo sapiens
  source 1..3348: mol_type = other RNA
accgtctcttctgttccccagacatgtcacatgaatgcaggtagctaggtacctgcgcgggctgttggttttgtaaacgcagagcagagcagtcacgatgtgtagaaatcatgcacctcagtgattctttaacaagataatgagtaaaaagacttcaggtatgtttgaaatgtctgccttttcctgcattctcatcactgacaaatatctgtgtagacattttactcaaatgtagacgtgctctttgcacacttgctagtacctgcctggtgcatttcaactgtgttttcttccaacagttgtacctcttagaagctgctgttttccatttggatctaaacactggacctgcacctgcgaccagctgtatattccaaaccactcctcggctttataaatctgacactgctcataatacattattcagaaaaggcatctctagtgtggctggccggctacgctttcacacatcagctaacacaggctatttctagagtgagtgcctcaaactggtctcctgggaccttttccttcgggaagagatccacatgttcttcacaggagaccagaaaaccagcacaacggccacgggtcctctgggcatgtaggtcttctctgtctcctcactagcacacactggcttgggtcattgtcacgcagtgcacacctttgtgccatgacaaagacacagggccaactcttccactatctccaagtctagtgtttgaacatttatgtacagacaaataaatgaaaaaaaaaaaaacataggcaacagaactccaaagcaaaacagaaactttggtcagatctattattccagttttgccagagaaaggctttccccaaatgtcgctgggtgagcgcggtcctatccccctacagctcctatcagccaacctggtggccttaacgttcatcactgtggactcaaaacacctaaaactgggaattttccaggcccagtttggcagtagggcttctgtaggcagtgaggtaagcggatcacacgttccgtggctgatctgtgtgagccgcagcttggtgctgggggacaccagcttcagctttgcaggaaagccatgtttaaagagtagcctccagtcctactggcccaatgcttttgccatcagggacctgacaaggtttagaatgaggtgagcgatggtgacagtatccctgggcctggacactgtgtgccaccctgactgtgtctggcagcccctccacctggctactgaagccagtcaggtgtgggggctgcagactgtccccctgccgtcaggtggctgaagggtccccagtgtgccagcatcagaggccaagttctctagctctctggtttgcagtttttagttttttttttttttttttaagatgaccacaagaagttttacattattatattcagacaaataaccatttagttactctatttcagagcactgaaaaaaacaagtagcaacagaagacagacttacaagggcactaagtctctggtcactcaaggaccaatcaaaggaatgcgctgttaggccagaaaggagtctctgaagcaaatgattggaaggaaaaaaaaaaaatctaaggaaatacaagccgaaaagtttccatttacaataaccaagggaaagagggacccgacatgatataaaatcccaaataagagctttccgctgaggcaggtttctgagcatggaaacaacaccggtagggactggaccggaccacagtctgcccaggccccgcctcggcccttctcgccgactccagcatgggaaatactctcatcgtcccggagcaaagatgaaatcaagagcctgccgttcggccgctgcgacgtttggatgccacaaatccaccatgaaaaccacccgtgggccatcctctgctgaaccttcatggaacgcagcatgcaggaaagagtcatcaaagagaaggcagcgcccttctgcccagcactggggctctccccccaccaccagctcacagccatttggagttttcagacctaaatggcatcggatgcggatgttggtgggtccatagtgctccgttatcacagtcccagggctcagcacagagatgcacgcgttcccaaaaacattgttcccaatacaggtccgaaggcttccgagcaagcggtacgtccgtgggcacttcctacagttcctgggaacacaaaccccctgattgaccaagtaaaaggtgaaccactccccgctgggggtgctgttcattttccatccttgcgggaggctgcagtttgagaaagctttgtagagggtctcaaactcacacaggatggtctggaagttccgttccagcacttccacatcatgtttctgtgcgtcccgggagaaatagggcgtggtgggcaggtcgggcaggaagaagacctcgggcttctggatggagggccggctgttgaggtaccggccctgctcgcggatgcccttgtggatgcggcccatgccggaccaggagtagcgcttggcgtactcctgcaggttgtggtacagcttctggttgaggccctcgttgtgggtgcagcgcacgcactcaggggactggcagtacacgtagccattctgcagcccgttggcatcggcagcctgcatgagggagttgacggagacgtagggccggggctgctccctgcccacgtgataacagtaccacacgaagaggaccaggaggcaggccacagtgatgacagcggtggtgtcgcagtcccgcacggactggatgccggtggcgatgcagtccctcaggccatccagcgaccagctccaggccaccagccactcgagcgacatcttgggggagtccttactgggcgtgtgaagcaaggtcagacaatcagtcctcgggggtcccaagggcgcccacaccatgcagattagcgtgggggggaaggagcggctggggcagggggaggcatggctgccaccgatcctcagatactgccaggggcggcattgatgaacgacaaggttggccgtgcccactgctccactttccggcaaaagtcactgcagtggggtggaagaggctggtttttgtcacattatcaagtgccgtcggtccctgtgaaaggatttgtttaggaaaaccaaacctgcgcccgggcgcgcggacggctgccgggacccaggagacgccgccgcccgagggcgcggacccgcggacggcccctgcccggcgccgcggagccgccgcctggctgctgcccagcccacgccgcgggagcccgagccggagcccgagcccgagcctaagccgcgccggtgcccctgccggtgccgacgccgcgctgcgctccgcggggccgcgaagaccacaact

SEQ ID NO: 8972 - RNA, 14607 nt, Homo sapiens
  source 1..14607: mol_type = other RNA
accgtctcttctgttccccagacattctcctggggcagagaaagaggccacagtgacatgacacactaatcacttctgcagcacaccaggaaccagatgcaccatcaaaaattctgctggtttccaggttgggcatatgaggaaaaagacaaaaagaattcttcacttcactgcttgaggccacacagtctctgtaacacactgaaggatgctaagttcctttggttttcctgcaaacaaccgctaacaccagtcttgtatttagagtaggatttaaaatccatccacagcccatactttttaaggaagcaaatcatggggttggcttcccatatgcttctcatctctggggtctgcttaccagttgacttctcatagcatgcttgccccgactgccttgcagtcttttcagatgaaattcaagattctccggtaactgtagcaggacaactcctaagatcagcgaccttccaaataaccttctcattcctctcatgttcagagaatgggaaaggatgccagaaagctatgtgagggtgaatgagggccagaattgtaatttatatctatgacctcggattcaagcattcatccagagtcatttgtcactgctaatgttttcccatggagttggatggcatgtgaagagaaaaatccctttaccctcctggaagaaatcttgagagttgactgctgtgtggtttgctgggaggttgtggtaaatgttgagaaccaccatctcataatcatatgcttgaagctttaaatcatgacttgaatatctgccatctctagatattggagtaggccctagaaaaaagcaaagatgaataatacatgattcccagtggaaagacagaaaagacctcatttgttacatgtggtatattgagtagtatgaaagatataaaaagtcacagtacactgcggaaactccccctgcgggaaaggcactgttttagcctctaggagtaacatacaggtcccaccttcaaggagctcacagtccaaaatcttgggtcatgcaaaaacctaatgccaactggtacaagccactaatcatgggcatctcatcatccaatcagcacacagctgtcacccctagtagaggatctttctagccccactgttctactttttcctggatgtcctcactgggattctggatagttctaatattaacagaacccctttgatctgagctctctgttctagactggaatcacttctgaggacttctttctggcctagataagcttgtctagaacaataactttcaaactgttatcagctgcgacccgtattaagaaatacgttttcatcagaactcagtctacatacatctgtgtttgtgtctgtgtgcagatgtacaaaaagctgattcaagtttcatgcaacaatgccttcatcatgacatgaaatgcactctgaattgtttgtgtactctatcctattttaaaatatttttgaatgtgctagttacaactcactatattgatttcatgacccactattgggttgcaacccacattttgtaaagaactggggaagtcccttaaagtgcgatccatggaccaacagcattgacattgcctgcgagtttgtcagaagtgaagaccctagaccaactgaatcagaatctgctcagattattgaggatcttttgaaactgcagattcagattcaataggtgtgaggtgggcctaagttctccatttctaacaagcttctgggtgacactgatgctgctaatattgagagcctactttgggtagcaaggatttaaagagaagacacaaagcagatggataaaattgaaatcactttttgaggctccactctgtaagttctgtgggggcagagatatatctatatagatcatcactgtatcccacgtgcctagtagattggctgacacacaatcagtgctcagtaaatgtagaattgattcattgagtagatggatgaaggaatgaataaattccagttaggctatagaatcaactcagtctctcatgtatatgctaaagtacaagtatcactgttggtgagaaaggtgagtcagatcaggaactcactccactgcctcaaccactaatgtagaggcaggcaactcaagaattcttaataaatagaaacatatttgctcacaaattaaactagcctcctatattggtttttgatttataaatagaaagaccatacagtttatcatccacatagagactccaagattaaaagagggccctgttaataaatcagactgcctggacatgcagagacatacaggtactctagaagcagtcaaaatactacagcttcaggtcaatatgggggaacataacgcccctcaaaccactttgtttatactttagtgatagcacttagcacattgtatcatggttgtttgcttaatgcctaggttcccaaatgcaatgtgagtacctgaaggccagggagggagttcacctctatgtctccagtgtcatctaggacctgtccactcagatgcaaaaaggtctattgaacagatttggtggtctagaaacacacaacctaccttagtaataggttatcttgactgtagccaacatagaaaaccagaagacattgggataaactgattcaaggagacttggtttcttttccctataataaaaaaagaatactaaaactctgatttcatgaaaaaaaaaatctcagtaacagtcaatgactgaaagaaagacaatgaagtagaggaacataggcaactaacgatctgtaggggatttgtggtagaaatgacagatgagagaatgccaagaaacaggatctagacagagttagctagcagccaagcaaaaatgcaggataattaataagtttcacattttcagaattggttaattgtgcacccagagattgttattactacaaccgatcattgcagatggcaaggccaggctatctgtaacttatcctacagccaaaatatcttggaggtactcctgactggcatctagccaaactgtgtcagttgaaggaagcttcatatctctaccatgtcagaatggaaccaactgccttttgagataaaacagcattcaaatagaaaacccttcaaaaaagaaaagacagaaataatttatggatccaaagatccaaacagttgatgtaaccacaggaattatttctcagatctacagggactgaaccattcctagtagatgttagcacagtgttgctgactgagttgggagtttatgcaggctcagtgctgaatccagagacgtgaatcactgaacaaatagctcaggttctctaatgggcaggtggtggcaccagttcactaaccagaaagagatgggaaggagggttaaagctgagctaatagtagctcccttaagacagcaaatcttctgcagaatatactccagtttgggcttcttattctggattttgagctgaatggtctgtgtgtcatcttttatgccttctcagcttagttcttaggagtttagaagagacagaaatggagtagaaagaaactaagaccatcattcagtaataacttaccttacggcaagtgccatattgtatcacctcatttaagattcagagccacactagaaattaggcatcatatacccaatttatatacagtaagccaagaggcagagaagttacttacagagaaggcaaagaagatttcatgtaagtgggaagttattgtgccaggcatctgaacttaggtctctctgaccccaaaactccatttgaaatttccccatagagtcagtggctctactgggaaagccctactcactccattccgccttggaatgatgtgcccttcaaacccagatggtacatgtcctgtgtgaactgcagaaataatacgtgagtaccctggaaacctgcagtttattatttctgtcttacacttaaaacacatggtggccacagtagttggaaacaaataagaggtgatctggtgctgggaaagtgagtaaccatgtaattagcaaagctaatgttgtgcagtttccataaataacatgctgtttacttttgttattaagagacttttaatattaaaaagtgtggggggtgtctaaggtagacaagaaagatgatatcaggcacctggcaaaggagggaaaaaacttactctgagaaactatctcttcattgtttaatgttctttacatccttaaaaataatcccctcagttttccttgcagcttgagaacttgattatttgttgcattggttatgagagtggtagagtgagacttccacctgaaaatttgcctacagagaagacagcttgttattattatccaagacagggagtctcctcatcaagattccaccccatggggtctgagccatggcagaagaggattaaagtgttagatcatgcagcacaagcagtccctcccagggttcttggaaatggctgcaaaccatctctaatctagacatttaagtctcctcccatatccttcattcctaactgcctgggtcaaactcattttctccttacctaatttttctgaaaatgcattattcaatatttctgttttggaagtattctcatctttttccattttgtggctttgctatctaatttcaaacataaatccactaagtagagttgacatctagttccagggtctgtccaggggactataggcatgcaataaatgttaaatcatgatgacaatagatacaaatagcaatgtgatcacagtgaaacacttcattttcctagttgcatgaactctacaaagctttgaccccaaaacagctttgtatgcacgtgtgtgtgcacgcacatgcacacacacacacgcacatgtttctatggtttctgttaccataggaagcatttccattctgctccattgtacgtttatacaacacctcattgctattgctatggtatccagaaacattgcttaaattaaatgaatagaaaacatcagggaagaagaaagggattaaaatacagacagttgaaagagaacagaataacagagggtaagaatgggtgatgatttttagaagcaattattttctaatgtaattttattctggtacatttctttttgaatacatatttcactgagcattctgattctcttcatccatgtaaaagcaacttggaggtatggaaaagagaccatatttctcagtcttaagatattcctgggaaggatatggagcccaggccaaatcatcctatgtgtttctcagcactgcccaagtgatgtatagttgaagaataaccttgaaagcaagaaattttcattaaatgccccccaaaaaagccaataataatgcctccatagcagataaggtgggtacaactgctattgctgattgcacagttgctgattaagagtctcaggtctttagcagcatcagctgatcatgccatcaagctcagtccacacactgtgccctgcttctccgccagctgaaatcttctgattctcttcctcagtctctcagacccagccagatttgaggctaaaagtttaactagctttctagccccatccttggtgccttcttcaagtcatgcttggtgccaacccagacctggtcttgtacaataattctgccattttctggtttgttccctggagttagagtaccaagttcctgtgtctgcttaatgtcccaagacattaagcaatacttacatgaggttctcaacatatttgacctaataatactaatagatgacatttgttcaatgccacctatgtggcacataaaatataaatgtatgtgccaggcaccactttccatgactgatcctgatacttacagatcaggaagttagctttttcagaatacccaaagcttcttaagcaatggacttgatttgaacccaattctgaggaaattagaatctaaatcaaattttaactttagtacattgaaaaattgtagccttacattagagcaatctgttaacatcaccaatagctggacaaattagcatgaggtgcatcctggtatgatgcactgagaacatagcatcacttcagtgtcattcctgcccaaagggtgtaacttcggtgcaatcatgaggaagcatcaggcaaactcaaattgagagacagtctgaaagacagttgacctatataccctttctaaaaatgtcaaaatgaaaaatcacaaagagaaactgttccagactaaaagagactaaagagacaactaactgcaacatgtaatttgattggtccctgaacatcccctcccaaaaccttttcattgggacaactggtgaaatacaagtttgtactttagatgttagcattgaatcagtattagttttctgattgcaataattataatgtgggtatatgagaatttactttttcttagaaaacacacaccaaagtatttgagcatgcaacttattctcaaatgattcataaaataataagtgtctatatagagagaaaattataaaaataaatgtggtaaaacattaacaattaggatattatagttggagggatatggaagttccctgtactcgtaactttttggagagtctaaaattatttcaaaataaaaaattaccaaacgattaattccatatagtagaagagtgtccttttcaggtatcagaagggtcaaatgacccatccacatcactagccattagcaaggcacctgagaagccaattaaattcaagagccagttgtacaactaatagtccctcagatcaattgctggtagaatgtcatgctgtccatctttctacatttaaccttatttcttcccattttcctcctctcttctctctttgttatgctcatgttttctagagcaccacattcaatgaactataaattaatgttctagagaaggagtgcagctcagtgaagagtggattgttggggtgcaatttccagctcttctgtttagtagcactgtatcccagggtaactgatctctaaaatgagtgtgataatactacttacctcatgaggttgttatgatgattacataaagtataaatgtaaggtgcctggcacatacatttatattttatgtgccacataggtggcattgaacaaatgccatctattagtattattaggtcaaatatgttaagaacttcataaataagttggcactatccttaatgagttcacatcacaaaggcacaaggggctagaattcaaaagggaatgtgaagtggagcaactatatagccatgactgaagtaagaaatgccccaaattcaaaataacaaaagacatgagcataaataagcaacttaattccattttagggctgtgacaaatctaaacaaagtggaaattacaggcaagagcagcaacagcttaaggaaaaatgaaacctaaaaacagttctttgcctcccaggggaagactttaaaaagatagggaagaatatttgaatatgagacaaaaacatgtgttactttctcatttcctgctcacgagatgctctgtctgccattatttaagctgtgtcgaggacatataatcagagactaagcagatataaatgctcaacaggatgattctttatgattccttggcaccctatgccaaacattaataaggtttgtgagaagccagtgagcactataaattgctctccttctaatatgaatcacgcgacagacttcatttgtttcctgcatgctgacctgacaatgagaaataaatctgataaagttctctaacttggaaaggatttgttttctgtccagggaatctatctcaataaggaaaaggttattgggcttcgagccacgggcaataatatgtatacctgaaccgctcctttggtattctgagcattgtcacacaggattccttgcttattcagcctttttaaatggtcccaaaggaatgtttttgtgcaagccgctcagcccacaaactcgcctgctgtgcatgatttaggactgaaatgtctttaagtgagccatattttactcgcaagggctgggtggccatcactttagatcctctgtcaccccaaactccatcgcttatttacatttttcatatttaaggggtaaatagttccaagacacatactccagttcataccttgtcagggtatcctgcaagcaggtcaaagaaaagggaattggcttcagcttgattttcgagtatttcagactgttttgcattctgacgctaatgatactcttcttaaaacagtagtgtgctgtattataattgcacataggcaaagtcataaccaacaactgtcaggaaggaaattttccatcttgtgaaaaaacataaataccagatgcttcagcactatattctcattttttttctaaaggactgaaattaaataaaactacacttagaagtaattagaaatccaagcaacgctctctatccaaaatggtgaggttctgttaataatattagtgatactcttttcttttaacacaaggatctcaaaatatatcctgaaaagctaaagaaaaagttgttaactaaataaattgtatataggacaataatcatagtgtccccacagagtctgattttttttttttttttttttgagagagagaggtcactctctgttacgcatgctggagtgcagtggccagaatctgaattttaatgcaaaagtaaaaactgtggcaattactgatgtatacaccaatactcctaataataattaaattcaagtcataggtaacatgtattgaatacttaatatatgccagccctgggctaagctctttatatggatagctgctttgagtcctcacttctaccctaagaaataagtataattattatcccccattctacagagaagtaaagtagagcttagcaggaggaaaatattccaccaaaggtcacagagcttatgttatagaggccgcattcaaacccaagtctctctccagagctgaagctcagccactttgccatacaacatctatcttcgaattctagcctatttctgcagcagcaaaaccctttccaacagcgcgagaagtagtgaggccaaaaagctagcaatttcttaaaagatccatctggaggctgggtgtggtgactcactcctgtaatcctagcactttgggaggccgaggcaggcagatcacttgaggccaggagttcgaaaccagcctggccaatatggtgaaaccctgtctctactaaaaatacaaaatattagccaggcatggtggcaggcgcctgtaatcccagctacttgggaggctgaggcaggagaatcacttgaacccaggaggcagaggttgcagtgagctgagatcataccactgcactccagcctgggtgacagaatgagactcaatcaaaaaaaaaaaaaatccaactggaatcctagtcaaaaaaacattaagatataaaaaataaggatgtcacatggaccaggagtggaaacggaaacaccaagatcccaattatggccagtagcccatctgttggatatcaaacaattatgtattgagcaccttccgtgggtctggcactattccaggcatttggatttgtgggagtaacccgactttggatttttccatattaattcaacacttttatcagaaacccaggtatcagtttctctgtactgggagccagggcctcaaagttaaatacacagcccctggtttcaaggaccttataatccagtgcaaacctcacagacaagaatcaggagtactttgctcttttacatggttgtgctttccccttactctcataccttctttcccctaaaaaatgaaagctaactctccatattgaaaatcaaacttttaagatacatcatgttggttttcataattaccctttaaaaagaagcaacaaggcaaaaaccatctcaatccatagaatcaaaatgcatgagagctaaaaaaaaaaaacaatcttaaagatcatgcatgctctgaggaaaccgaggcctccgtctccgaacaactgggggagctgtgcctctaccccgcatcatctggcttccaggtacttggttcttccccagtgcaccatgttgagctacctcctgcgtgatcaacccacgtcccttctgactgccagaaaaatgaaaagttttattgttcataattttggataaattgcaatattgtaggttcatataaattcactcacaaattacactcaataaaccccagtgagcaatttaaaggcatgataccaccccgtctcttgctgggagggcaaggtgatgatggagcaggagggaggagaatgaagaaagctcataaattaagagaagcaaaggagtgatttcatcaaagtgccaagctcagtccatggaatgtttcaattgtataaaatttataatgttctgagggggatgatttacgggtcctaatttttcacaataaaaagctcagtggggattctgtgaatgaaatatcttttttaaaataaattaaaaatgtagtttgaaatgagggtcagtggtgccacgtctggagaataactccttatcggatcagctccaaaaatgagtcacaggagaaaggccccataaaacatgtattatttaaaaaggcataggaaggtgtatgacaaataagcaatatgcagaaaagcatatctgatccaatttgtcccatcaataggataatatctttatcattaggtttcaatgaaaaaagaagaactcgatagaaatctaagggttttcatgaagattaaggtctttaaacaatgggagaagaagagaaaggaaggcataaaaatgaaatcttataaataagtaaatgtgtctcatatttaggaaaaaacaaaatgtaaatatgtactgcttcctgcaaatttgacctatatggaattagaacctaaatgtcatgcaataattcttagacccttccttcagtgaggtcttctacaaggagaacattaagagcttcccctctgtccacaggtgcagccaaatgatagtcctataaatggggacaggcccactgagccacaatcctacattaactgggcccacctgtatgttggtccatccattcttcacagctgtggctcaacctcagcttcctgatagtgactgaatccttcaagaggctatattcctgttcctccaggttgggttcttgaccaactacctggactttccagtttctctctctgaaaggcttactgaaccccagtcctagtacacccagtttcttgccacccactcctgactagttggccttgtatctcagctccggcaagagtaaagcttgagttgactacatcactttgaacggcgactattcatagcaagttatctccctcaatacacacctcctagttgatgctttatctcctgggctccatctccacaagccaaacctgctgtttagccaagattattcaaattttgatggtgattatttagtagttgaaacaaggagatcagaatcagttttctaaatttgtaagtgctatttttaatttcctaagtgaaatataattgtctcaaatctttgtacatttcttgcttctttcatttctgtggtggataggctccaaggtggtccccccatgaccccagattcttgttgttcatgcccttgtataaccccatctccttcagattaggtaagacttgtgacttgcttccaatcaacagaatatagcaaaggagataggaagtcactctcattatgacattatgttatgtaagactccatcttaccagcaaatttgctccaaagactctctctcagtagctgtcttgaagaagaaaattgccattttgtaaaaaggcatatgagagacaaccttgtagcatggacctggggtggaaggggcagccaataattgctgagaaaggcttaatctgatagctagcaagaagctggagccctcagtcttacaaccacaaggaaatgacttttgccaacaacctaagtgagtttggaagcagaaccatctccacttgagcctccagatgagaactgagcctcaactaacacgttgattgcaactttgaagaggaccagttaagacatgcccaacacctgacctacagaattgtaattacagaaatatatgtgtgttgttttaagccactatgtctgtggaaatttgttaagcagcaatatataacctatacaactttaactcaaataaatacaaagacaactcaattgtgcattgtggtgaatagtataaaagactcacttttaatcctttagacacagccagaaacaagaaggagtttacaatctggatggaaagattaaacaaaattaaacaatatcatatgacaaatgagaattagcgtaggaccatttatgatcaattgccaaatacatgaggcaggcataaattctccaagtatgctgtgggaagagaagtcactgggtcccaggaagagtttacgatggaagtcgaggaggttccacagttcttgcaggataaatagagcctgctttggcagagatgaggagtaacacatttgagacaggaaatagaaaacaacacactctgatctctgtagaaatgaaaatgccattctctatgggatgaacaattatataagacaacaattatatgactttggcaaattattttctctctctaaacctcagttccctctgctgtaatacaggaaaagtaatggtatcatcctcagtaagttgttttgaaagtccaataacagaattaaagtgcttagcacagtaagaacctgatacatgtttgctattattattgccagtagaacttttttatacttactagaagagagtgcagttcagtaaaagaactgccattataccagaccctttaagtcagctcagagtcaaggtaagagtctcagcctcttctctgggccattccaaggacacattgccctcagttcctgcttcctgccttcctgcctagcattgttaggcacttttacgacaataaagattctcatactaaatcactgggcaacttgagaacaaagggcttgtttatttcatcttcttaactctcaccaggtccaaaacaaagcttggcatctagtaaatcctcctgaagtggtttgcttttgtgttttttcaacgacgaggccagcatcgcaggaggctggggactgcggtgggtggcaaagataaagatattgctcaaaattcatcctatgtcctttgaagtgttttgcttaaggtcttggaatttaatcccaccctgtccagcttcaggcgaatttttctggcccagttaatatagttagttcaaactttatttaatatagggttggctaccatggacacattcttttcttcttttctttcagagttcatctcaagagatgttccttgtttgcaagtctctccacaataactgattgccatgatcagcagcaacctgaggaggtcccattcatttgtatgtttgcaagctgcactgcctccatggagagagcacccatcccctctcttgcaccaaaaattcaaatttagaacgcactacatctatcggcatttataaacatgaggcatatgtgagtcttctggttagctgatggtatttacagtcttcctgttgttcagcactgacactggaacataagtcccaggagtttactggaatattcacatatggtcaaatattaaggcatcttggtatatttgagatgcagtgtgttttcacacagacaattggcatctggcttgaatgttgaaaggtatggagggaaacggagatgccaataggaaatcaaaagaacagaagagcatgaagaatggcctttctctcaaccaaaagagaactggaaatgcggcagcttcctcagatgatcagctgtccacgtctgaaaattcagtgtgcctccagggtattttcacttaaaattaatccagaatgttgtttccagctgtgtgtccttgggcaaactgcataacctctctgcacattggtttcatcatctataaaaatgggaacagatacacctgatgctttactgcattgggtagttgtgattctgattaatatgaagtaacatatatagtcttataaaatatagaatagtattactattagcttcattgaatcattttgcaagtggaatatatataattaatttcaaagttattattaattgtagtaaacaatttcttgtctgcctaagagcacgtcttttctgggaactgccccctcgactatctccctcccagtccagacttcatcagctttgtaggagtctccatgttgaataacaagggttctctacccctgggccacagaccagtacctgtccttggcctgttaggaaccagtccgcacagcaggaagtgagcagtgtgcttcatctgtatttataactgctccccactgctcacattacccctgagtaatgtgagtaacctctacctcctgtcagatcagcagtggcattaggttctcatggaagcgtgaaccccactgtgaaccgtgcatagaaggcatctaggttgcatgctccttatgagaatcaaatgcctgatgatctgtcactgtctcacatcacccccacaggagacctgtctagttgcagaaaaacaagctgagatctcccactgattctacattatggtgggttgtataattatttcatta

SEQ ID NO: 8973 - RNA, 51 nt, Homo sapiens
  source 1..51: mol_type = other RNA
accgtctcttctgttccccagccccttctttactgtcgtcctctgggggca

SEQ ID NO: 8974 - RNA, 435 nt, Homo sapiens
  source 1..435: mol_type = other RNA
accgtctcttctgttccccagccccttctttactgtcgtcctctgggggcacatccatgttatcggactctgcctgctcgctgctacccttttcctgctcgtctatccagtcggacacagctttgagcgcccgctccgtgtgggacaccatgttctggactgcctccagctcctcttgtgttggataaacggaagaatgctttgccatcacatggcggtcatcattcacaaaaattcgcattggacgcatttttacttcttctgtagtgtctggaaatcaaacttttgcttatcttttcaaattgtgatagagttccttggtgttatcaatacttcaactccacaaaggcttcctcagcaatccgcgtgggaaggggcttccaaggagggggtccgcctctccgcgacctgtgaggacaaaggaggcgacttttc

SEQ ID NO: 8975 - RNA, 600 nt, Homo sapiens
  source 1..600: mol_type = other RNA
accgtctcttctgttccccagccccttctttactgtcgtcctctgggggcacatccatgttatcggactctgcctgctcgctgctacccttttcctgctcgtctatccagtcggacacagctttgagcgcccgctccgtgtgggacaccatgttctggactgcctccagctcctcttgtgttggataaacggaagaatgctttgccatcacatggcggtcatcattcacaaaaattcgcattggacgcatttttacttcttctgtagtgtctggaaatcaaacttttgcttatcttttcaaattgtgatagagttccttggtgttatcaatacttcaactccacaaaggcttcctcagcaatccgcgtgggaaggggcttccaaggagggggtccgcctctccgcgacctgtgaggacaaaggaggcgacttttcccgcctcgggaacctgggactctcctggaatcgggggcgggaccgggacaaagaggaggagggggtagggaaggagtgaggaaggggggtcgccccgccgcggaactcgggacccgagggggtgtgtgctccaagcacgtgcgcgcgtccccaggacccccgcaa

SEQ ID NO: 8976 - RNA, 458 nt, Homo sapiens
  source 1..458: mol_type = other RNA
accgtctcttctgttccccagccccttctttactgtcgtcctctgggggcacatccatgttatcggactctgcctgctcgctgctacccttttcctgctcgtctatccagtcggacacagctttgagcgcccgctccgtgtgggacaccatgttctggactgcctccagctcctcttgtgttggataaacggaagaatgctttgccatcacatggcggtcatcattcacaaaaattcgcattggacgcatttttacttcttctgtagtgtctggaaatcaaacttttgcttatcttttcaaattgtgatagagttccttggtgttatcaatacttcaactcttgtcggcgtccccttcttcgaccgcagccgccgccgccgccctcctgccacagcccgccggggtctgcccccaaaagccacgcggtgcgcgccgggctgctgggtccaactgcaat

SEQ ID NO: 8977 - RNA, 482 nt, Homo sapiens
  source 1..482: mol_type = other RNA
accgtctcttctgttccccagccccttctttactgtcgtcctctgggggcacatccatgttatcggactctgcctgctcgctgctacccttttcctgctcgtctatccagtcggacacagctttgagcgcccgctccgtgtgggacaccatgttctggactgcctccagctcctcttgtgttggataaacggaagaatgctttgccatcacatggcggtcatcattcacaaaaattcgcattggacgcatttttacttcttctgtagtgtctggaaatcaaacttttgcttatcttttcaaattgtgatagagttccttggtgttatcaatacttcaactcttgtcggcgtccccttcttcgaccgcagccgccgccgccgccctcctgccacagcccgccggggtctgcccccaaaagccacgcggtgcgcgccgggctgctgggtccaactgcaatggcgagaagaggaggaggaggagt

SEQ ID NO: 8978 - RNA, 691 nt, Homo sapiens
  source 1..691: mol_type = other RNA
accgtctcttctgttccccagccccttctttactgtcgtcctctgggggcacatccatgttatcggactctgcctgctcgctgctacccttttcctgctcgtctatccagtcggacacagctttgagcgcccgctccgtgtgggacaccatgttctggactgcctccagctcctcttgtgttggataaacggaagaatgctttgccatcacatggcggtcatcattcacaaaaattcgcattggacgcatttttacttcttctgtagtgtctggaaatcaaacttttgcttatcttttcaaattgtgatagagttccttggtgttatcaatacttcaacttgaaagcagctcccgggagaagtggaccgtaatctgcagcaggggatataccaagtgagcctggatcctaccggagcgccagaaagcaacaaagcactggtgactatagcagtcttgtcctgaggacatcggagctgacttgtgaggtgtcccactggcttgtcggcgtccccttcttcgaccgcagccgccgccgccgccctcctgccacagcccgccggggtctgcccccaaaagccacgcggtgcgcgccgggctgctgggtccaactgcaatggcgagaagaggaggaggaggagtccggaccgggggcgagcgggcgggcgggcaggcgcgcgccggggaggtgcg

SEQ ID NO: 8979 - RNA, 999 nt, Homo sapiens
  source 1..999: mol_type = other RNA
acctcgccgtcccgcccgccgaggcagccgccgccgccgagccgccgccgccgcccgcagggggcgcccgggtgctgcccccgctggccgcgccccgccgctgccggcggctgccgcgaccgcagtcgtcgccgccgcgctcctgccaggcggacttggagcggaagctgaagccgaagcccccggccagggggtcgtcaccgctcagcggaggatcgtcgtcgtcgtcgctgcgccagcggctggccaggcgctgctgctgctgcggggtcaccgcccccccgggtttcttggtggagccgcgggcagagcccccgggggcatgggggtagccattcgcgcgggaatcggcctcgccccacgcagagcggtgttcggggcctccccggggcgccggcgccgcagtcttctgcgccgcgtagcccggggggctcacgcttttggagccggacatccccccctcggcctcgtcgtctccttcctcctcccccggaagccgggccgggggtctccaaggggagggcggacggccgagcagggggaccaggctagggtcacacgtcgggggcggcccggggccctgcgctgcagcggggcatcttggcacccccgtcctgagcggaggaggagggcacagccccgaggtgagaagtagctgaggatccgcgtcagaagtcccaggtccgaaatggagttgcctccgaggtggggtcgcagggactggtctggctgctgctgcgccgcacgcggagagacgtccgggatcctggctcgcgtcgagctcgacgagggccggagttgcggacgagacgggacggagtggtgtccttgcgggcggtgcctcctcgggccggcagtgcccgggcgcggcgctcgctgattccgcctaagcggagcccagctgctctcggggctcggcggcggcgagggcggctcggcgggggtcccggcgaagagacactgcgggtgcgctttcctcgcagcggactgggagcgact

SEQ ID NO: 8980 - RNA, 3533 nt, Homo sapiens
  source 1..3533: mol_type = other RNA
acctcgccgtcccgcccgccgccttctgcgtcgcggggcgggccggcggggtcctctgacgcggcagacagccctcgctgtcgcctccagtggttgtcgacttgcgggcggcccccctccgcggcggtgggggtgccgtcccgccggcccgtcgtgctgccctctcggggggtttgcgcgagcgtcggctccgcctgggcccttgcggtgctcctggagcgctccgggttgtccctcaggtgcccgaggccgaacggtggtgtgtcgttcccgcccccggcgccccctcctccggtcgccgccgcggtgtccgcgcgtgggtcctgagggagctcgtcggtgtggggttcgaggcggtttgagtgagacgagacgagacgcgcccctcccacgcggggaagggcgcccgcctgctctcggtgagcgcacgtcccgtgctcccctctggcgggtgcgcgcgggccgtgtgagcgatcgcggtgggttcgggccggtgtgacgcgtgcgccggccggccgccgaggggctgccgttctgcctccgaccggtcgtgtgtgggttgacttcggaggcgctctgcctcggaaggaaggaggtgggtggacgggggggcctggtggggttgcgcgcacgcgcgcaccggccgggcccccgccctgaacgcgaacgctcgaggtggccgcgcgcaggtgtttcctcgtaccgcagggccccctcccttccccaggcgtccctcggcgcctctgcgggcccgaggaggagcggctggcgggtggggggagtgtgacccaccctcggtgagaaaagccttctctagcgatctgagaggcgtgccttgggggtaccggatcccccgggccgccgcctctgtctctgcctccgttatggtagcgctgccgtagcgacccgctcgcagaggaccctcctccgcttccccctcgacggggttgggggggagaagcgagggttccgccggccaccgcggtggtggccgagtgcggctcgtcgcctactgtggcccgcgcctcccccttccgagtcgggggaggatcccgccgggccgggcccggcgttcccagcgggttgggacgcggcggccggcgggcggtgggtgtgcgcgcccggcgctctgtccggcgcgtgaccccctccgccgcgagtcggctctccgcccgctcccgtgccgagtcgtgaccggtgccgacgaccgcgtttgcgtggcacggggtcgggcccgcctggccctgggaaagcgtcccacggtgggggcgcgccggtctcccggagcgggaccgggtcggaggatggacgagaatcacgagcgacggtggtgcgggcgtgtcgggttcgtggctgcggtcgctccggggcccccggtggcggggccccggggctcgcgaggcggttctcggtgggggccgagggccgtccggcgtcccaggcggggcgccgcgggaccgccctcgtgtctgtggcggtgggatcccgcggccgtgttttcctggtggcccggccgtgcctgaggtttctccccgagccgccgcctctgcgggctcccgggtgcccttgccctcgcggtccccggccctcgcccgtctgtgccctcttccccgcccgccgcccgccgatcctcttcttccccccgagcggctcaccggcttcacgtccgttggtggccccgcctgggaccgaacccggcaccgcctcgtggggcgccgccgccggccactgatcggcccggcgtccgcgtcccccggcgcgcgccttggggaccgggtcggtggcgccccgcgtggggcccggtgggcttcccggagggttccgggggtcggcctgcggcgcgtgcgggggaggagacggttccgggggaccggccgcgactgcggcggcggtggtgggggcagccgcggggatcgccgagggccggtcggccgccccgggtgccgcgcggtgccgccggcggcggtgaggccccgcgcgtgtgtcccggccgcggtcggccgcgctcgaggggtccccgtggcgtccccttccccgccggccgcctttctcgcgccttccccgtcgccccggcctcgcccgtggtctctcgtcttctcccggcccgctcttccgaaccgggtcggcgcgtcccccgggtgcgcctcgcttcccgggcctgccgcggcccttccccgaggcgtccgtcccgggcgtcggcgtcggggagagcccgtcctccccgcgtggcgtcgccccgttcggcgcgcgcgtgcgcccgagcgcggcccggtggtccctgccggacaggcgttcgtgcgacgtgtggcgtgggtcgacctccgccttgccggtcgctcgccctttccccgggtcggggggtggggcccgggccggggcctcggccccggtcgcggtcccccgtcccgggcgggggcgggcgcgccggccggcctcggtcggccctcccttggccgtcgtgtggcgtgtgccacccctgcgcccgcgcccgccggcggggctcggagccgggcttcggccgggccccgggccctcgaccggaccggtgcgcgggcgctgcggccgcacggcgcgactgtccccgggccgggcaccgcggtccgcctctcgctcgccgcccggacgtcggggccgccccgcggggcgggcggagcgccgtccccgcctcgccgccgcccgcgggcgccggccgcgcgcgcgcgcgcgtggccgccggtccctcccggccgccgggcgcgggtcgggccgtccgcctcctcgcgggcgggcgcgacgaagaagcgtcgcgggtctgtggcgcggggccccggtggtcgtgtcgcgtggggggcgggtggttggggcgtccggttcgccgcgccccgccccggccccaccggtcccggccgccgcccccgcgcccgctcgctccctcccgtccgcccgtccgcggcccgtccgtccgtccgtcgtcctcctcgcttgcggggcgccgggcccgtcctcgcgaggccccccggccggccgtccggccgcgtcggggcctcgccgcgctctaccttacctacctggttgatcggttctcggcggcgtcgcggcgggtctgggggggtctcggtgccctcctccccgccggggcccgtcgtccggccccgccgcgccggctccccgtcttcggggccggccggattcccgtcgcctccgccgcgccgctccgcgccgccgggcacggccccgctcgctctccccggccttcccgctagggcgtctcgagggtcgggggccggacgccggtcccctcccccgcctcctcgtccgcccccccgccgtccaggtacccggcggccgtcgcgcgcctgccgcgcgtgtggcgtgcgccccgcgccgtgggggcgggaacccccgggcgcctgtggggtggtgtccgcgctcgcccccgcgtgggcggcgcgcgcctccccgtggtgtgaaaccttccgacccctctccggagtccggtcccgtttgctgtctcgtctggccggcctgaggcaaccccctctcctattgatcat

SEQ ID NO: 8981 - RNA, 84 nt, Homo sapiens
  source 1..84: mol_type = other RNA
acctcgccgtcccgcccgccgtccgccgtccgccgtccgcccggccctcgccccctcccgagctgtccagcgcagccgccctct

SEQ ID NO: 8982 - RNA, 432 nt, Homo sapiens
  source 1..432: mol_type = other RNA
acctgccagcacctccctgcagcagtgcctttgcacctgctgtttccttatcctggaatgctctcctcaggtggccacgactcactccctcacttcccttatataaaatccctgatctctgctcagcatcagattccagtggccttccctcatctctctaaagcagcagcctccaccccaacacaggctatcccctccccagctcacgtctctccatagcacctagtcccttctgtatcatgtgccggtctgatttctctaactccgcaccctagatgtgagcttcttgagagctgaacttccacagctgaattcctagcatctcaagcttgcctggctcaggggaggcattcataagcatgcgctgaataagggaaggaattctgtccaaggagcatctgctatatatcctgccttctaaggcacagtgag

SEQ ID NO: 8983 - RNA, 4821 nt, Homo sapiens
  source 1..4821: mol_type = other RNA
accttcctctccatgggtcttttgcatttctccatgtcttttgagtagaactattgactgccctttgttcaaggctgtcttttcaaggatgtttacacagcaaacagccctggaagatatagtgtctctttccaggccaaagggcaggcatgcttacggcctattacaaaaaattcaggttccctacacatggtgttctcttctgtagcaaaatccagaaagtgagctggcatttatctggcctcctgcatcacttctggggaactcagaggaaaggggaagtgacttaaatatgctaacactcatttagcgtgctgttctgtaagtaagaaaatctgagctgtcttgtgtcttctgccagggtatgagaaactgtgacaagcctacttgtaagtttacaaataaggtaaaatataaaacccttcacagttcttgacactgccatgctacttcaatgtttcaaacatgtaaatctaatagccccaactagattatgcttcattaatcctacaattcattcagtgcctagttttgcagagtgacagttctataaaaatctcattgaataatacttcaacatattttgagaaacaaaacagaaaggaaagaggttatctctcatgtttatgaaaccctatgatcaaggaaaggcttcttgagaaattgggtaatgtctgaaagttaagaataaggctaaactcagagggctagagaaagatccaaaatgaaacaatcactgagaacccatctctagatctgatttctgaatctgtgctgcacactgatactgcctaatctgaaagcagcctgcatcattatcatcctcaccacctccaacaaattacttacttctctagtgtgcctacttggtcttaagaaggatgtaactgtcatggtgacagcacagttgaacttcaggaattagaaaagcagcaacacagagcttctctaagccttgaactgaggcaggtgggccacagttaacagtcatccggctatgggcttccaaacagctgtggaccactcgggcatgagcaagaagcctgcataatgagtctatgcaggagctagggtaaggcacagctgtcaagtagaaggtcgcacactagagcattgtgccacacaagaagttcaacattcaccggaaaaaaaaaattgtttaatatcccacttagaatgacctctacctacctgtatttatttagaaagtgaaatctgtagcactgttcaccccagaagctctggaaagagtatttctatagttactgaattaacctcgccagcattccacaggtgatctggggtaaaatacataacctcagtcatttaagagaaaacaccaatggaatgatggcacttgattcataagtggtaaagtccaaatttgacaaatcaaaactgttcttgaccagaaactttaaattccaaacgtcaagtgaactaatttgaactaaatgtcaaatttttttctagccttcttcttccctgacatttttaatttcacacgacaattttggatgtcatcatgctgagtctcatcacccatcagaacatttaaattaaagacatctgacagacagatttggcttatgaattcattttcataatgttcaaatatctgtgtctgacaagtgggcttttttgtaataagcatattataagccagcaggagtcatcttgctagttacattttcatgcaagaattagatattagaagattcctaggtcagtgcaatcaactgcaatttaaacatttttaaaggacttatcagcttttagaaaaggactatcgtgacttccaaatgggaccagaaatggcagaaaagaaaagcaatgtatcatgatatttttcctatatccttatgcccttcatcttaaaacttgtaactgaaatataaaaggtggttaaaataacggtttatgaaatatgtattctacagggattttttttcctcttcccttcaacaagggctgcaactgaaaatcagcaaagttttatcttgctcgcttcattcccaacctcaggcaaactctcaaccccaagctcctcttttgctgccgatactccacaacttaccgcaagtggattctccaggtctctgtgcctcctctccagtcctctatcccagacttccagggtgtagtcacaccccatgattaataattccatggtatggagtaaacatcaagcattttgcacattattcttctgagtccaaaaaaatgtacctcatcacaagcttcctaagaaggatttcgttaataccagaaggtttttctaattgtcacctaacttagtccctggacataacatgtgctcaatcaatggctttttaactgaactaattataacaattttcagcagatcaagagcagagatattgtggttcacaaacattttacaacacaggcacagggcctgatagacactgactgatcaattctgcggggagagagagagaaagagaccatacataatattttactcaataaatgtacaagaaaatttgagccattttatcttcatgagaaattcttcagatcaaataacagaatcatgataataaccataaaataatacaattttaggcatttacaatgcaccatatattatcatcatcatgttatatacattgcttctgcgctgggctataccacatatattagtcaggttatgtgagttaatgctacaaatacagccctgaaatctcagacacttcaatcaaacagcaaaggcttttttctgcctcatgttatatggccattggtggccagctggggctgacagagcaccatgtcaacccttgattccacgattcccaagtcaggagaaaggatgtgacaatgacaactagtacactggtttgcaaaggcttctgcctaaaaaagacacacagcgtttcaaaaagcccttcaaacctcaaaaatcactcaaaaaattgagcatataatggaacctaggaagttctttaaataaagctcttaaaatgacaacaaaggattaaagtaactggactgtccaatagcaaatacaatacattaaaattgcaatggtagcaaaacgtatcacacgttttctatgtacaaggtatcattctgacgtttaacaggtactagctcatttaatcctcaggacagccttttaaggtaggtacgaatactatctccatttgactgacaaggtaactgaggaaccaagaggttgaataaattgcccaagggcacacagctgttaagtagtaaacaagagactggaaatagacattctggctacaacgtctgtacactgaacctctgtcaatctaaaccattgcaatacatgtgaagactttgttggttaaatttcagtatgaataaatatacacaataatctacaattacacaattcctgtctagttttaatttccagttctttcagtaatgtgtgccttgaagaaaatgttcctggcctatctggtcttttctgttttgtctgttattcttggtaagttcctgtggggcagagatcacactaacatccagcaacatgacagcaacataattaatgcttaataaatatttgtggagcaaatgaataaaattcaagttttccatttcttctgacttatcaatctgactcataacatctaaactagaaagtgcttttattacttttttaatgttaatgcatattttaaaaacctttgagttcctggtctgcaaaattcaaacatagtcattatcaattgctaatttctgtcaacgtactctcaaaattctggccatgtatgttgcccaagaaatagcttgttggtatcaattgcacaaatattcttctgatctcccccatgctgtttaaccatttggtactatgtcctgtagcctgcatgagcaccctacagcatcctgagcagaaggccctgagtgcacaagaagaaattcagttgcctattatacacaaattccccaccgcccctcatgtcttcctcactgtccagaatccagacttggagataatagataacaggtcagagaaatctgataccaagcgtaagattcaaaaaactcatcattttatgtagaaatctatactgaaaattcttttttcctttgatgtattgatcactgactgcaacaaaataagcagaagtgagacataaggagataataatggagaaaaaaagagactgcaaaacagactactatactaaagactgtagtccatattggaaaagagaccgtctcatgattgcccctctggctgttacattaagtacctagtttcctatatgaactttgctttacatactaataggatgttcttaaagatttgaaataagccacaggcctaggagagtattccttgaactgtactccattgatttgcttttcctgaaatgcctgtatatccttgatgttaaatgggttctttgatcaaatagactagaaaaaaaatggatccaggataattacgtcagtttctttgttcagactgctcagctacttttcaatgcacacaattgtataaatagaaacctctaaggtatgttcattatattttcccatctttgtgcaccaccatgatgaaatagcctatgcttttgaacatctatacttgtatagaaaatgtatctttgtagaatcatatttgacaagtaaagtctttctttcaaatccgtggctgatgacttaaatgttcccaaagcccttatagttgaggacccacgtgtcaaataagcatggcattttaactcagtcctaagcacacactgtgtacacacacacacacatacacacacacacacacacacacacacacacacacacacagagatcagtaaa

SEQ ID NO: 8984 - RNA, 6621 nt, Homo sapiens
  source 1..6621: mol_type = other RNA
accttcttgtataagcactgtgctaaacactgaatcctcacaaaaccctaagtgctaagaaagctagggtaatttttttctgcattcaagactctacagctaatttggtcttttgctataaaaacttggtctcccactttttgttgaagcgaacaagaatcacaggaactcaccctcagcttcacgaaactcccagcttcctaaatgagcatgaatctatttatgtccatccgtctactcacatgaagatgctctgcagctccacagggatggatgggattagaataaagccaatatggaaattaaaatacttttaaataaataaaataatccaggcttgggatagtaacacatacaacagagcctgtcgttaacaaaatagacttttctttttaaatcaagaatttttggccagaggtgagggtggcaatgtctaatatacacaagctaggtaaaccaccttggagaaatggggtggccaccgtggtctgccctaaaaggcacacacctacctacagacatacagtttcagtccaacacatcatactgatgtcaaccctgtcagtgagctgcactgggctccactcccaaaggggaagctcattattcacttttattaaatcttgcattcactaaagaaacaaaaaaggggtgcacgttctttccctttcatgatgctaaagtatttcttctccaagcagggccctgaactccttggatgcacccattcacatgattctgcctcagccacacctcagcaagtgcgtgggtggcagggaacacaggctggttgacacgttggcaaccagcagtcccaaggtagacccaaaggtatggcagaatccagccctttcttgaggttctcaaggcttcacaccctcctctgtgggtggaagtgcacatgcatacacgctatggcctggcgggggggttatagggagcgtctggtgtccagcttcaacagctacagtggctcaagaacatgtcctgtctcttagctggaggagtctgctattgcccttcaacagcatccggattccaaaaaccccaaagaaaaacgaaaaggcacatcaaggaaacaaatatcactaaagaaactgactaatatctccaaacgcacagcaaacacacaaaaaagcaaactgtaatgagcagtgacacaaacccagtccaaacaaaaatgaaaagcatctccatttatacatgtgcaaatcaaactgcatacacaaaataaatgcggtgtttaccagcattcaaagaagtctttttactcctcaaagtatctacctttcaatggaaagctttctcttttagtaaattagatgaatgttttccctcaagttttttaagagcttaggatcacaatggggaaaataatccaaaaaaacaggcaagatattatagcggggaaaaacattaatcataacttaggatttctctccccatggaactgttatcagctataaatcggtttaggattctatcaagatcagcaatggcaaaacctccgcaggcttccagcccacacaggggcaccttcctctcctcttccatgcagggcagttggaagccccctccccagtttcctctccaggatcactgactagacctgggccaagtctgaggaggcctgggagccagtacacattcaggggtcactgactcttcagataatgccctaaacaactggagtgtgggcttgtttgctccaagagcagctgccctgtcagtggaactccggcgcacttccactcaatactggactgggggggatgaaagagggatttttaaatggcagaaaagtgttcttctgggctgtctggcccgggcagggcgggttgtgacttggaaaagaaggggaaggtagggaggccttgaacttagggacagccagcaaatgatccttgcagcttttggaacacaaggcagggctaaggttacctttcagcttccttgcttaagtagcagtggctaagtgggttaaactttgctcggcctgcaggctccccctgttggtcagatacttgcattgacatcctcagtgttcaatgctcctggaagagcccaggagagggcggcactggcccagggattgcaggtcagggaactctagcaaattcccacaccctagggtacagccaagaggcccattcacaaggaaaaagctcttccttacagcaaggatgccagtcatctgccctcctactgcaggaaactgcccttgcttaaaagaaatgcacaggctcatacacacacacacacacacacacacacacacacacacacacacacacactcactcaccaaggtttcctttggacttctgcccttcttcctaggcccaagcagaggctattctcagccaggtctggaggcgcccctgtgatgatgctcagggcagaggcctccccatggtactctacctggcagatgtgcttgggggccacctaaggagtggaggaggccccgggtgccccccaccctcctcttagactggagatacaattgagacgcactgagcagggatctcagtgggcctaagaaaaaaggctggctgcacatttgtgtagcaattgagaaagaagcagaatgtaacttcccagacttaaaggccccacactaactctagtccccatgaagcggaattcttcctttccctcacattctgaaagctaccagccattacgccttgcccatcagttctgcccagcggaggctccactgggccgccctctgttagcaggaagggtgcttggaagccccggcacagagcacatcattgagcgactgaggcgcccagcagaggccaagtggaggacgccaaccgctcacattaggcagaaggggtctcacttgcatcagcatggagatgtcaggggcttttcagaaacttacaaacttgtacagagcatggcagcaatgattcagtggggtgggaacttatacaaaggcagagcatgggggggtccagggtttggaaggtggggtccagtgtgtctgaccaggccaacctgatgactgattactcaacaagtcagagtgatcctgcctgaaggaaaagccagcaccagattcccacctttgcgagctacaccctcaggtgagtagccaggacagggcactgcattcatcctgagctgcccccactcccccagcagacatcaagagcccccttccctggactttggtgccatcagaggggacacaacacaagcccacctgtcaggagcccagctccggtcgcgccacaaattcttaaggaccgacttcactcctgtccaaatcttggctcaaagataatcctctccaagtccatgaacagcgtgagtctttcatctctactttcctcctcatagcggggctggagggagggtgagtttaccagaaactccaaaatccctcaatcctgtatttccttcccaaagggattctaaaagaaattacggccaaggtatgtgtctgggcatggggacatggaggaaaggggcctcatctcctttttcgtccctggctgggctctctggacaacacaggcacgtccccctgactgaggcagcccatgctctaggtgccatctatgacgatgccctggggagtttggctgtgcttccaaagcaaaagtttcttttgttctgctgccatctgttttgagctgccaggtccccatggctgtccctgagcaggccaccagccccacggcacacggtctctctcctgcaccctgcccaaagcagacagaacaacagtatagtgaaggtggatgattaacagtggaaataaaagaagcctgtgatcaatccctcctctccctcccgcggtcccctccctcccacccgaataaataagttaatgggtttaggaatattcccattcagagttctttcccatcagctcaattcctcctgttttgttttaaaggactcttgagactttcttttgccctggagcagctgcagtgacagtcttcccacagttgctccttgagaaacagaaatgatgttgtgccagggacaagccaggctcctggcctgacatacgctcttgttttgttttggtgaagactccactgggttgctcggagtgcagcaagggcaatgccaattcagaaccttctacgaaaaagttcaggctcttgccagagtccctgcatgacttctgtccctggccctgcctgacggggctggggccactgtcttccccagcagcatggtgcagggctgagcaggtagctgctataggcagtctttgcagagagccacctggcccttgatgaagtcccggcaggggcagaccctctggtgcctggggtgggcgcctgcacagctgaagagcaggaggtcaccttgaaacacacagtgcttattcttagggtcaaaggagggcaccaggatgtccttggccagctctgagctttggcaggtcaccttgtacttcagcatgtccttgtccttgttgaggtgctggaagaaagaaggctcgcagatgagctggctctcctggcacacctgcttgcaggactgcccgggctcagcaagcttgacctgtagggcgctgaggggtggccacatcacttgcccatggcagaagtcctgtttttcaatgaaagcattgattctctgtagcatcccctcgcacgtaaattcatatggcatgtatggctcaatcttctgatttaaaattgctttcactgcatcctctacttcctcctgattgttgaggtcaacagtccacacatgtggccgcccgatgaaaacttcagcgtaaggatgctgggatgtcagctctctcagagttggcttgccaatgaaaaagtctgtgtttttgctgcttttgggtgggttgaacttgggattcagaaaagcacatccatttgcgatagcttccaggggagctgggccctcgtaagggaacccaagtccaacaaacaacttggtttctcgaagaaggaactgcaggtcccgtccactgaggataccatggtttttcacgtaactgggaatattctttgtgctggagccataaacagttgcatgcacttccatgtatgtgtgaataatgtccaagtagatcttcttattcttccagaagctatccactttgccatacacaagggactggttctgccttttgatttcattaatgtggtggatatcactggagttcaggtgctgctcaaccacaaaccccagaaagctgttgtctggggtatgagggaacatggtataaaactgctgagggttcagattccattttccccaaggggtcttgtggcctttcgattgggcataatttgcatgattaaattcgggttcagtaccaaatgaatcaaggactcggagcatgcactggtaatgaacccaggatggtccaagagttttcttgaattgagcaagtcctacaatatcaatgtaaatgagctcaacaattctgtctcctacagttgggcagccagatcggtttcctacaaccttcttcatgatttccttgagctcagccagtgaagctgaaatcctaatgtcatggcccagtaagtacagagatgtaattaaatcactccattgaactaattcaccaagagggccaccactgaaagctgtctctgcaatcttaaatccagattccttggtcaggagtcccaggtgaacgaggactttcttccgctttctcttttcaaggttctgcttttctgccagggacttgattgcttggatccatgcgtcagccattcgccggatccgtagtctcatccaccggaattcttcatgctttttcatcatactgtagagaatattaaaatctgtacgaatttccgccaatgaattatgatcagcttcttcgtagggattttttgctctccaaggtaaatgaggacaccaattttcaacctcactgaggtaaataaaaaaagagcaggtggatccatccactccatagtctgcgtagcagggatctgaacgccacatgtctttcatccacttgatctttccctcacagtgagggtagccgtccataggaggcaatacacatttttcttgagctccgttaatgatatctgccacattaattttctcaagtgcaaccaagctgggaacagctgtagtggagttggttgagtttgttccggtgccattgacaacaagattgtccaccttcgactccaacttgccaatgcgctgcaaaatgttatctaataacacagcaagggttttcttcagatcataagctgtcatgactccagcgtatggcccatccaccacattcctgttttcttctgccagtgccttgatgtaccttttgctgaggtccaggatctgctcgcgcagcatggagctgctttcaggctgagttcgctgctggatggtaaagtgcagaagcatcataccccaaatgaagccaaaagtcaccaggaaaaagcccagcttctgagaggacaacttccacggagtgaagagagccattgctctctggcaacttcacctgtccttggctcttaacgcgtagaagatagacacaaattcatggtgtaggttgagtgtgagagtctgctggtctcactctggctcctgtgtcagctggttgcctttcctcacttccattaagcaacatgatccatttcccgtc

SEQ ID NO: 8985 - RNA, 6817 nt, Homo sapiens
  source 1..6817: mol_type = other RNA
accttcttgtataagcactgtgctaaacactgaatcctcacaaaaccctaagtgctaagaaagctagggtaatttttttctgcattcaagactctacagctaatttggtcttttgctataaaaacttggtctcccactttttgttgaagcgaacaagaatcacaggaactcaccctcagcttcacgaaactcccagcttcctaaatgagcatgaatctatttatgtccatccgtctactcacatgaagatgctctgcagctccacagggatggatgggattagaataaagccaatatggaaattaaaatacttttaaataaataaaataatccaggcttgggatagtaacacatacaacagagcctgtcgttaacaaaatagacttttctttttaaatcaagaatttttggccagaggtgagggtggcaatgtctaatatacacaagctaggtaaaccaccttggagaaatggggtggccaccgtggtctgccctaaaaggcacacacctacctacagacatacagtttcagtccaacacatcatactgatgtcaaccctgtcagtgagctgcactgggctccactcccaaaggggaagctcattattcacttttattaaatcttgcattcactaaagaaacaaaaaaggggtgcacgttctttccctttcatgatgctaaagtatttcttctccaagcagggccctgaactccttggatgcacccattcacatgattctgcctcagccacacctcagcaagtgcgtgggtggcagggaacacaggctggttgacacgttggcaaccagcagtcccaaggtagacccaaaggtatggcagaatccagccctttcttgaggttctcaaggcttcacaccctcctctgtgggtggaagtgcacatgcatacacgctatggcctggcgggggggttatagggagcgtctggtgtccagcttcaacagctacagtggctcaagaacatgtcctgtctcttagctggaggagtctgctattgcccttcaacagcatccggattccaaaaaccccaaagaaaaacgaaaaggcacatcaaggaaacaaatatcactaaagaaactgactaatatctccaaacgcacagcaaacacacaaaaaagcaaactgtaatgagcagtgacacaaacccagtccaaacaaaaatgaaaagcatctccatttatacatgtgcaaatcaaactgcatacacaaaataaatgcggtgtttaccagcattcaaagaagtctttttactcctcaaagtatctacctttcaatggaaagctttctcttttagtaaattagatgaatgttttccctcaagttttttaagagcttaggatcacaatggggaaaataatccaaaaaaacaggcaagatattatagcggggaaaaacattaatcataacttaggatttctctccccatggaactgttatcagctataaatcggtttaggattctatcaagatcagcaatggcaaaacctccgcaggcttccagcccacacaggggcaccttcctctcctcttccatgcagggcagttggaagccccctccccagtttcctctccaggatcactgactagacctgggccaagtctgaggaggcctgggagccagtacacattcaggggtcactgactcttcagataatgccctaaacaactggagtgtgggcttgtttgctccaagagcagctgccctgtcagtggaactccggcgcacttccactcaatactggactgggggggatgaaagagggatttttaaatggcagaaaagtgttcttctgggctgtctggcccgggcagggcgggttgtgacttggaaaagaaggggaaggtagggaggccttgaacttagggacagccagcaaatgatccttgcagcttttggaacacaaggcagggctaaggttacctttcagcttccttgcttaagtagcagtggctaagtgggttaaactttgctcggcctgcaggctccccctgttggtcagatacttgcattgacatcctcagtgttcaatgctcctggaagagcccaggagagggcggcactggcccagggattgcaggtcagggaactctagcaaattcccacaccctagggtacagccaagaggcccattcacaaggaaaaagctcttccttacagcaaggatgccagtcatctgccctcctactgcaggaaactgcccttgcttaaaagaaatgcacaggctcatacacacacacacacacacacacacacacacacacacacacacacacactcactcaccaaggtttcctttggacttctgcccttcttcctaggcccaagcagaggctattctcagccaggtctggaggcgcccctgtgatgatgctcagggcagaggcctccccatggtactctacctggcagatgtgcttgggggccacctaaggagtggaggaggccccgggtgccccccaccctcctcttagactggagatacaattgagacgcactgagcagggatctcagtgggcctaagaaaaaaggctggctgcacatttgtgtagcaattgagaaagaagcagaatgtaacttcccagacttaaaggccccacactaactctagtccccatgaagcggaattcttcctttccctcacattctgaaagctaccagccattacgccttgcccatcagttctgcccagcggaggctccactgggccgccctctgttagcaggaagggtgcttggaagccccggcacagagcacatcattgagcgactgaggcgcccagcagaggccaagtggaggacgccaaccgctcacattaggcagaaggggtctcacttgcatcagcatggagatgtcaggggcttttcagaaacttacaaacttgtacagagcatggcagcaatgattcagtggggtgggaacttatacaaaggcagagcatgggggggtccagggtttggaaggtggggtccagtgtgtctgaccaggccaacctgatgactgattactcaacaagtcagagtgatcctgcctgaaggaaaagccagcaccagattcccacctttgcgagctacaccctcaggtgagtagccaggacagggcactgcattcatcctgagctgcccccactcccccagcagacatcaagagcccccttccctggactttggtgccatcagaggggacacaacacaagcccacctgtcaggagcccagctccggtcgcgccacaaattcttaaggaccgacttcactcctgtccaaatcttggctcaaagataatcctctccaagtccatgaacagcgtgagtctttcatctctactttcctcctcatagcggggctggagggagggtgagtttaccagaaactccaaaatccctcaatcctgtatttccttcccaaagggattctaaaagaaattacggccaaggtatgtgtctgggcatggggacatggaggaaaggggcctcatctcctttttcgtccctggctgggctctctggacaacacaggcacgtccccctgactgaggcagcccatgctctaggtgccatctatgacgatgccctggggagtttggctgtgcttccaaagcaaaagtttcttttgttctgctgccatctgttttgagctgccaggtccccatggctgtccctgagcaggccaccagccccacggcacacggtctctctcctgcaccctgcccaaagcagacagaacaacagtatagtgaaggtggatgattaacagtggaaataaaagaagcctgtgatcaatccctcctctccctcccgcggtcccctccctcccacccgaataaataagttaatgggtttaggaatattcccattcagagttctttcccatcagctcaattcctcctgttttgttttaaaggactcttgagactttcttttgccctggagcagctgcagtgacagtcttcccacagttgctccttgagaaacagaaatgatgttgtgccagggacaagccaggctcctggcctgacatacgctcttgttttgttttggtgaagactccactgggttgctcggagtgcagcaagggcaatgccaattcagaaccttctacgaaaaagttcaggctcttgccagagtccctgcatgacttctgtccctggccctgcctgacggggctggggccactgtcttccccagcagcatggtgcagggctgagcaggtagctgctataggcagtctttgcagagagccacctggcccttgatgaagtcccggcaggggcagaccctctggtgcctggggtgggcgcctgcacagctgaagagcaggaggtcaccttgaaacacacagtgcttattcttagggtcaaaggagggcaccaggatgtccttggccagctctgagctttggcaggtcaccttgtacttcagcatgtccttgtccttgttgaggtgctggaagaaagaaggctcgcagatgagctggctctcctggcacacctgcttgcaggactgcccgggctcagcaagcttgacctgtagggcgctgaggggtggccacatcacttgcccatggcagaagtcctgtttttcaatgaaagcattgattctctgtagcatcccctcgcacgtaaattcatatggcatgtatggctcaatcttctgatttaaaattgctttcactgcatcctctacttcctcctgattgttgaggtcaacagtccacacatgtggccgcccgatgaaaacttcagcgtaaggatgctgggatgtcagctctctcagagttggcttgccaatgaaaaagtctgtgtttttgctgcttttgggtgggttgaacttgggattcagaaaagcacatccatttgcgatagcttccaggggagctgggccctcgtaagggaacccaagtccaacaaacaacttggtttctcgaagaaggaactgcaggtcccgtccactgaggataccatggtttttcacgtaactgggaatattctttgtgctggagccataaacagttgcatgcacttccatgtatgtgtgaataatgtccaagtagatcttcttattcttccagaagctatccactttgccatacacaagggactggttctgccttttgatttcattaatgtggtggatatcactggagttcaggtgctgctcaaccacaaaccccagaaagctgttgtctggggtatgagggaacatggtataaaactgctgagggttcagattccattttccccaaggggtcttgtggcctttcgattgggcataatttgcatgattaaattcgggttcagtaccaaatgaatcaaggactcggagcatgcactggtaatgaacccaggatggtccaagagttttcttgaattgagcaagtcctacaatatcaatgtaaatgagctcaacaattctgtctcctacagttgggcagccagatcggtttcctacaaccttcttcatgatttccttgagctcagccagtgaagctgaaatcctaatgtcatggcccagtaagtacagagatgtaattaaatcactccattgaactaattcaccaagagggccaccactgaaagctgtctctgcaatcttaaatccagattccttggtcaggagtcccaggtgaacgaggactttcttccgctttctcttttcaaggttctgcttttctgccagggacttgattgcttggatccatgcgtcagccattcgccggatccgtagtctcatccaccggaattcttcatgctttttcatcatactgtagagaatattaaaatctgtacgaatttccgccaatgaattatgatcagcttcttcgtagggattttttgctctccaaggtaaatgaggacaccaattttcaacctcactgaggtaaataaaaaaagagcaggtggatccatccactccatagtctgcgtagcagggatctgaacgccacatgtctttcatccacttgatctttccctcacagtgagggtagccgtccataggaggcaatacacatttttcttgagctccgttaatgatatctgccacattaattttctcaagtgcaaccaagctgggaacagctgtagtggagttggttgagtttgttccggtgccattgacaacaagattgtccaccttcgactccaacttgccaatgcgctgcaaaatgttatctaataacacagcaagggttttcttcagatcataagctgtcatgactccagcgtatggcccatccaccacattcctgttttcttctgccagtgccttgatgtaccttttgctgaggtccaggatctgctcgcgcagcatggagctgctttcaggctgagttcgctgctggatggtaaagtgcagaagcatcataccccaaatgaagccaaaagtcaccaggaaaaagcccagcttctgagaggacaacttccacggagtgaagagagccattgctctctggcaacttcacctgtccttggctcttaacgcgtagaagatagacacaaattcatggtgtaggttgagtgtgagagtctgctggtctcactctggctcctgtgtcagctggttgcctttcctcacttccattatgcttcagtcaaaggattcttctttgcaagcggcccaaaagaaaatggtagcaggatcttgaagcaattagctttcagagccctggatcactgttggtctgcctcttactgttttcccattgccttgttccttcccactgacgcctcaacacaacaaaatcatcttcaacctttataaagatggttagagatctctggcaaagaaatgtgtcaattctc

SEQ ID NO: 8986 - RNA, 6721 nt, Homo sapiens
  source 1..6721: mol_type = other RNA
accttcttgtataagcactgtgctaaacactgaatcctcacaaaaccctaagtgctaagaaagctagggtaatttttttctgcattcaagactctacagctaatttggtcttttgctataaaaacttggtctcccactttttgttgaagcgaacaagaatcacaggaactcaccctcagcttcacgaaactcccagcttcctaaatgagcatgaatctatttatgtccatccgtctactcacatgaagatgctctgcagctccacagggatggatgggattagaataaagccaatatggaaattaaaatacttttaaataaataaaataatccaggcttgggatagtaacacatacaacagagcctgtcgttaacaaaatagacttttctttttaaatcaagaatttttggccagaggtgagggtggcaatgtctaatatacacaagctaggtaaaccaccttggagaaatggggtggccaccgtggtctgccctaaaaggcacacacctacctacagacatacagtttcagtccaacacatcatactgatgtcaaccctgtcagtgagctgcactgggctccactcccaaaggggaagctcattattcacttttattaaatcttgcattcactaaagaaacaaaaaaggggtgcacgttctttccctttcatgatgctaaagtatttcttctccaagcagggccctgaactccttggatgcacccattcacatgattctgcctcagccacacctcagcaagtgcgtgggtggcagggaacacaggctggttgacacgttggcaaccagcagtcccaaggtagacccaaaggtatggcagaatccagccctttcttgaggttctcaaggcttcacaccctcctctgtgggtggaagtgcacatgcatacacgctatggcctggcgggggggttatagggagcgtctggtgtccagcttcaacagctacagtggctcaagaacatgtcctgtctcttagctggaggagtctgctattgcccttcaacagcatccggattccaaaaaccccaaagaaaaacgaaaaggcacatcaaggaaacaaatatcactaaagaaactgactaatatctccaaacgcacagcaaacacacaaaaaagcaaactgtaatgagcagtgacacaaacccagtccaaacaaaaatgaaaagcatctccatttatacatgtgcaaatcaaactgcatacacaaaataaatgcggtgtttaccagcattcaaagaagtctttttactcctcaaagtatctacctttcaatggaaagctttctcttttagtaaattagatgaatgttttccctcaagttttttaagagcttaggatcacaatggggaaaataatccaaaaaaacaggcaagatattatagcggggaaaaacattaatcataacttaggatttctctccccatggaactgttatcagctataaatcggtttaggattctatcaagatcagcaatggcaaaacctccgcaggcttccagcccacacaggggcaccttcctctcctcttccatgcagggcagttggaagccccctccccagtttcctctccaggatcactgactagacctgggccaagtctgaggaggcctgggagccagtacacattcaggggtcactgactcttcagataatgccctaaacaactggagtgtgggcttgtttgctccaagagcagctgccctgtcagtggaactccggcgcacttccactcaatactggactgggggggatgaaagagggatttttaaatggcagaaaagtgttcttctgggctgtctggcccgggcagggcgggttgtgacttggaaaagaaggggaaggtagggaggccttgaacttagggacagccagcaaatgatccttgcagcttttggaacacaaggcagggctaaggttacctttcagcttccttgcttaagtagcagtggctaagtgggttaaactttgctcggcctgcaggctccccctgttggtcagatacttgcattgacatcctcagtgttcaatgctcctggaagagcccaggagagggcggcactggcccagggattgcaggtcagggaactctagcaaattcccacaccctagggtacagccaagaggcccattcacaaggaaaaagctcttccttacagcaaggatgccagtcatctgccctcctactgcaggaaactgcccttgcttaaaagaaatgcacaggctcatacacacacacacacacacacacacacacacacacacacacacacacactcactcaccaaggtttcctttggacttctgcccttcttcctaggcccaagcagaggctattctcagccaggtctggaggcgcccctgtgatgatgctcagggcagaggcctccccatggtactctacctggcagatgtgcttgggggccacctaaggagtggaggaggccccgggtgccccccaccctcctcttagactggagatacaattgagacgcactgagcagggatctcagtgggcctaagaaaaaaggctggctgcacatttgtgtagcaattgagaaagaagcagaatgtaacttcccagacttaaaggccccacactaactctagtccccatgaagcggaattcttcctttccctcacattctgaaagctaccagccattacgccttgcccatcagttctgcccagcggaggctccactgggccgccctctgttagcaggaagggtgcttggaagccccggcacagagcacatcattgagcgactgaggcgcccagcagaggccaagtggaggacgccaaccgctcacattaggcagaaggggtctcacttgcatcagcatggagatgtcaggggcttttcagaaacttacaaacttgtacagagcatggcagcaatgattcagtggggtgggaacttatacaaaggcagagcatgggggggtccagggtttggaaggtggggtccagtgtgtctgaccaggccaacctgatgactgattactcaacaagtcagagtgatcctgcctgaaggaaaagccagcaccagattcccacctttgcgagctacaccctcaggtgagtagccaggacagggcactgcattcatcctgagctgcccccactcccccagcagacatcaagagcccccttccctggactttggtgccatcagaggggacacaacacaagcccacctgtcaggagcccagctccggtcgcgccacaaattcttaaggaccgacttcactcctgtccaaatcttggctcaaagataatcctctccaagtccatgaacagcgtgagtctttcatctctactttcctcctcatagcggggctggagggagggtgagtttaccagaaactccaaaatccctcaatcctgtatttccttcccaaagggattctaaaagaaattacggccaaggtatgtgtctgggcatggggacatggaggaaaggggcctcatctcctttttcgtccctggctgggctctctggacaacacaggcacgtccccctgactgaggcagcccatgctctaggtgccatctatgacgatgccctggggagtttggctgtgcttccaaagcaaaagtttcttttgttctgctgccatctgttttgagctgccaggtccccatggctgtccctgagcaggccaccagccccacggcacacggtctctctcctgcaccctgcccaaagcagacagaacaacagtatagtgaaggtggatgattaacagtggaaataaaagaagcctgtgatcaatccctcctctccctcccgcggtcccctccctcccacccgaataaataagttaatgggtttaggaatattcccattcagagttctttcccatcagctcaattcctcctgttttgttttaaaggactcttgagactttcttttgccctggagcagctgcagtgacagtcttcccacagttgctccttgagaaacagaaatgatgttgtgccagggacaagccaggctcctggcctgacatacgctcttgttttgttttggtgaagactccactgggttgctcggagtgcagcaagggcaatgccaattcagaaccttctacgaaaaagttcaggctcttgccagagtccctgcatgacttctgtccctggccctgcctgacggggctggggccactgtcttccccagcagcatggtgcagggctgagcaggtagctgctataggcagtctttgcagagagccacctggcccttgatgaagtcccggcaggggcagaccctctggtgcctggggtgggcgcctgcacagctgaagagcaggaggtcaccttgaaacacacagtgcttattcttagggtcaaaggagggcaccaggatgtccttggccagctctgagctttggcaggtcaccttgtacttcagcatgtccttgtccttgttgaggtgctggaagaaagaaggctcgcagatgagctggctctcctggcacacctgcttgcaggactgcccgggctcagcaagcttgacctgtagggcgctgaggggtggccacatcacttgcccatggcagaagtcctgtttttcaatgaaagcattgattctctgtagcatcccctcgcacgtaaattcatatggcatgtatggctcaatcttctgatttaaaattgctttcactgcatcctctacttcctcctgattgttgaggtcaacagtccacacatgtggccgcccgatgaaaacttcagcgtaaggatgctgggatgtcagctctctcagagttggcttgccaatgaaaaagtctgtgtttttgctgcttttgggtgggttgaacttgggattcagaaaagcacatccatttgcgatagcttccaggggagctgggccctcgtaagggaacccaagtccaacaaacaacttggtttctcgaagaaggaactgcaggtcccgtccactgaggataccatggtttttcacgtaactgggaatattctttgtgctggagccataaacagttgcatgcacttccatgtatgtgtgaataatgtccaagtagatcttcttattcttccagaagctatccactttgccatacacaagggactggttctgccttttgatttcattaatgtggtggatatcactggagttcaggtgctgctcaaccacaaaccccagaaagctgttgtctggggtatgagggaacatggtataaaactgctgagggttcagattccattttccccaaggggtcttgtggcctttcgattgggcataatttgcatgattaaattcgggttcagtaccaaatgaatcaaggactcggagcatgcactggtaatgaacccaggatggtccaagagttttcttgaattgagcaagtcctacaatatcaatgtaaatgagctcaacaattctgtctcctacagttgggcagccagatcggtttcctacaaccttcttcatgatttccttgagctcagccagtgaagctgaaatcctaatgtcatggcccagtaagtacagagatgtaattaaatcactccattgaactaattcaccaagagggccaccactgaaagctgtctctgcaatcttaaatccagattccttggtcaggagtcccaggtgaacgaggactttcttccgctttctcttttcaaggttctgcttttctgccagggacttgattgcttggatccatgcgtcagccattcgccggatccgtagtctcatccaccggaattcttcatgctttttcatcatactgtagagaatattaaaatctgtacgaatttccgccaatgaattatgatcagcttcttcgtagggattttttgctctccaaggtaaatgaggacaccaattttcaacctcactgaggtaaataaaaaaagagcaggtggatccatccactccatagtctgcgtagcagggatctgaacgccacatgtctttcatccacttgatctttccctcacagtgagggtagccgtccataggaggcaatacacatttttcttgagctccgttaatgatatctgccacattaattttctcaagtgcaaccaagctgggaacagctgtagtggagttggttgagtttgttccggtgccattgacaacaagattgtccaccttcgactccaacttgccaatgcgctgcaaaatgttatctaataacacagcaagggttttcttcagatcataagctgtcatgactccagcgtatggcccatccaccacattcctgttttcttctgccagtgccttgatgtaccttttgctgaggtccaggatctgctcgcgcagcatggagctgctttcaggctgagttcgctgctggatggtaaagtgcagaagcatcataccccaaatgaagccaaaagtcaccaggaaaaagcccagcttctgagaggacaacttccacggagtgaagagagccattgctctctggcaacttcacctgtccttggctcttaacgcgtagaagatagacacaaattcatggtgtaggttgagtgtgagagtctgctggtctcactctggctcctgtgtcagctggttgcctttcctcacttccattcacaagcctgcccatcaccagattgcaagtcttcagtggccaagaacttcagatgcataaagcagaaagacagcctgcccatccacaagccagcaccccatgtccatccaaagttggggtgcat

SEQ ID NO: 8987 - RNA, 6966 nt, Homo sapiens
  source 1..6966: mol_type = other RNA
accttcttgtataagcactgtgctaaacactgaatcctcacaaaaccctaagtgctaagaaagctagggtaatttttttctgcattcaagactctacagctaatttggtcttttgctataaaaacttggtctcccactttttgttgaagcgaacaagaatcacaggaactcaccctcagcttcacgaaactcccagcttcctaaatgagcatgaatctatttatgtccatccgtctactcacatgaagatgctctgcagctccacagggatggatgggattagaataaagccaatatggaaattaaaatacttttaaataaataaaataatccaggcttgggatagtaacacatacaacagagcctgtcgttaacaaaatagacttttctttttaaatcaagaatttttggccagaggtgagggtggcaatgtctaatatacacaagctaggtaaaccaccttggagaaatggggtggccaccgtggtctgccctaaaaggcacacacctacctacagacatacagtttcagtccaacacatcatactgatgtcaaccctgtcagtgagctgcactgggctccactcccaaaggggaagctcattattcacttttattaaatcttgcattcactaaagaaacaaaaaaggggtgcacgttctttccctttcatgatgctaaagtatttcttctccaagcagggccctgaactccttggatgcacccattcacatgattctgcctcagccacacctcagcaagtgcgtgggtggcagggaacacaggctggttgacacgttggcaaccagcagtcccaaggtagacccaaaggtatggcagaatccagccctttcttgaggttctcaaggcttcacaccctcctctgtgggtggaagtgcacatgcatacacgctatggcctggcgggggggttatagggagcgtctggtgtccagcttcaacagctacagtggctcaagaacatgtcctgtctcttagctggaggagtctgctattgcccttcaacagcatccggattccaaaaaccccaaagaaaaacgaaaaggcacatcaaggaaacaaatatcactaaagaaactgactaatatctccaaacgcacagcaaacacacaaaaaagcaaactgtaatgagcagtgacacaaacccagtccaaacaaaaatgaaaagcatctccatttatacatgtgcaaatcaaactgcatacacaaaataaatgcggtgtttaccagcattcaaagaagtctttttactcctcaaagtatctacctttcaatggaaagctttctcttttagtaaattagatgaatgttttccctcaagttttttaagagcttaggatcacaatggggaaaataatccaaaaaaacaggcaagatattatagcggggaaaaacattaatcataacttaggatttctctccccatggaactgttatcagctataaatcggtttaggattctatcaagatcagcaatggcaaaacctccgcaggcttccagcccacacaggggcaccttcctctcctcttccatgcagggcagttggaagccccctccccagtttcctctccaggatcactgactagacctgggccaagtctgaggaggcctgggagccagtacacattcaggggtcactgactcttcagataatgccctaaacaactggagtgtgggcttgtttgctccaagagcagctgccctgtcagtggaactccggcgcacttccactcaatactggactgggggggatgaaagagggatttttaaatggcagaaaagtgttcttctgggctgtctggcccgggcagggcgggttgtgacttggaaaagaaggggaaggtagggaggccttgaacttagggacagccagcaaatgatccttgcagcttttggaacacaaggcagggctaaggttacctttcagcttccttgcttaagtagcagtggctaagtgggttaaactttgctcggcctgcaggctccccctgttggtcagatacttgcattgacatcctcagtgttcaatgctcctggaagagcccaggagagggcggcactggcccagggattgcaggtcagggaactctagcaaattcccacaccctagggtacagccaagaggcccattcacaaggaaaaagctcttccttacagcaaggatgccagtcatctgccctcctactgcaggaaactgcccttgcttaaaagaaatgcacaggctcatacacacacacacacacacacacacacacacacacacacacacacacactcactcaccaaggtttcctttggacttctgcccttcttcctaggcccaagcagaggctattctcagccaggtctggaggcgcccctgtgatgatgctcagggcagaggcctccccatggtactctacctggcagatgtgcttgggggccacctaaggagtggaggaggccccgggtgccccccaccctcctcttagactggagatacaattgagacgcactgagcagggatctcagtgggcctaagaaaaaaggctggctgcacatttgtgtagcaattgagaaagaagcagaatgtaacttcccagacttaaaggccccacactaactctagtccccatgaagcggaattcttcctttccctcacattctgaaagctaccagccattacgccttgcccatcagttctgcccagcggaggctccactgggccgccctctgttagcaggaagggtgcttggaagccccggcacagagcacatcattgagcgactgaggcgcccagcagaggccaagtggaggacgccaaccgctcacattaggcagaaggggtctcacttgcatcagcatggagatgtcaggggcttttcagaaacttacaaacttgtacagagcatggcagcaatgattcagtggggtgggaacttatacaaaggcagagcatgggggggtccagggtttggaaggtggggtccagtgtgtctgaccaggccaacctgatgactgattactcaacaagtcagagtgatcctgcctgaaggaaaagccagcaccagattcccacctttgcgagctacaccctcaggtgagtagccaggacagggcactgcattcatcctgagctgcccccactcccccagcagacatcaagagcccccttccctggactttggtgccatcagaggggacacaacacaagcccacctgtcaggagcccagctccggtcgcgccacaaattcttaaggaccgacttcactcctgtccaaatcttggctcaaagataatcctctccaagtccatgaacagcgtgagtctttcatctctactttcctcctcatagcggggctggagggagggtgagtttaccagaaactccaaaatccctcaatcctgtatttccttcccaaagggattctaaaagaaattacggccaaggtatgtgtctgggcatggggacatggaggaaaggggcctcatctcctttttcgtccctggctgggctctctggacaacacaggcacgtccccctgactgaggcagcccatgctctaggtgccatctatgacgatgccctggggagtttggctgtgcttccaaagcaaaagtttcttttgttctgctgccatctgttttgagctgccaggtccccatggctgtccctgagcaggccaccagccccacggcacacggtctctctcctgcaccctgcccaaagcagacagaacaacagtatagtgaaggtggatgattaacagtggaaataaaagaagcctgtgatcaatccctcctctccctcccgcggtcccctccctcccacccgaataaataagttaatgggtttaggaatattcccattcagagttctttcccatcagctcaattcctcctgttttgttttaaaggactcttgagactttcttttgccctggagcagctgcagtgacagtcttcccacagttgctccttgagaaacagaaatgatgttgtgccagggacaagccaggctcctggcctgacatacgctcttgttttgttttggtgaagactccactgggttgctcggagtgcagcaagggcaatgccaattcagaaccttctacgaaaaagttcaggctcttgccagagtccctgcatgacttctgtccctggccctgcctgacggggctggggccactgtcttccccagcagcatggtgcagggctgagcaggtagctgctataggcagtctttgcagagagccacctggcccttgatgaagtcccggcaggggcagaccctctggtgcctggggtgggcgcctgcacagctgaagagcaggaggtcaccttgaaacacacagtgcttattcttagggtcaaaggagggcaccaggatgtccttggccagctctgagctttggcaggtcaccttgtacttcagcatgtccttgtccttgttgaggtgctggaagaaagaaggctcgcagatgagctggctctcctggcacacctgcttgcaggactgcccgggctcagcaagcttgacctgtagggcgctgaggggtggccacatcacttgcccatggcagaagtcctgtttttcaatgaaagcattgattctctgtagcatcccctcgcacgtaaattcatatggcatgtatggctcaatcttctgatttaaaattgctttcactgcatcctctacttcctcctgattgttgaggtcaacagtccacacatgtggccgcccgatgaaaacttcagcgtaaggatgctgggatgtcagctctctcagagttggcttgccaatgaaaaagtctgtgtttttgctgcttttgggtgggttgaacttgggattcagaaaagcacatccatttgcgatagcttccaggggagctgggccctcgtaagggaacccaagtccaacaaacaacttggtttctcgaagaaggaactgcaggtcccgtccactgaggataccatggtttttcacgtaactgggaatattctttgtgctggagccataaacagttgcatgcacttccatgtatgtgtgaataatgtccaagtagatcttcttattcttccagaagctatccactttgccatacacaagggactggttctgccttttgatttcattaatgtggtggatatcactggagttcaggtgctgctcaaccacaaaccccagaaagctgttgtctggggtatgagggaacatggtataaaactgctgagggttcagattccattttccccaaggggtcttgtggcctttcgattgggcataatttgcatgattaaattcgggttcagtaccaaatgaatcaaggactcggagcatgcactggtaatgaacccaggatggtccaagagttttcttgaattgagcaagtcctacaatatcaatgtaaatgagctcaacaattctgtctcctacagttgggcagccagatcggtttcctacaaccttcttcatgatttccttgagctcagccagtgaagctgaaatcctaatgtcatggcccagtaagtacagagatgtaattaaatcactccattgaactaattcaccaagagggccaccactgaaagctgtctctgcaatcttaaatccagattccttggtcaggagtcccaggtgaacgaggactttcttccgctttctcttttcaaggttctgcttttctgccagggacttgattgcttggatccatgcgtcagccattcgccggatccgtagtctcatccaccggaattcttcatgctttttcatcatactgtagagaatattaaaatctgtacgaatttccgccaatgaattatgatcagcttcttcgtagggattttttgctctccaaggtaaatgaggacaccaattttcaacctcactgaggtaaataaaaaaagagcaggtggatccatccactccatagtctgcgtagcagggatctgaacgccacatgtctttcatccacttgatctttccctcacagtgagggtagccgtccataggaggcaatacacatttttcttgagctccgttaatgatatctgccacattaattttctcaagtgcaaccaagctgggaacagctgtagtggagttggttgagtttgttccggtgccattgacaacaagattgtccaccttcgactccaacttgccaatgcgctgcaaaatgttatctaataacacagcaagggttttcttcagatcataagctgtcatgactccagcgtatggcccatccaccacattcctgttttcttctgccagtgccttgatgtaccttttgctgaggtccaggatctgctcgcgcagcatggagctgctttcaggctgagttcgctgctggatggtaaagtgcagaagcatcataccccaaatgaagccaaaagtcaccaggaaaaagcccagcttctgagaggacaacttccacggagtgaagagagccattgctctctggcaacttcacctgtccttggctcttaacgcgtagaagatagacacaaattcatggtgtaggttgagtgtgagagtctgctggtctcactctggctcctgtgtcagctggttgcctttcctcacttccattctccttgttgggcagcagcagcagccgggagcacccgccggccgccgtgcccacgcggcccgaggcgcgaggtcgcgacgccccgagcctgcggcgcggctacctgggctggatcgcgcccggggccgccgccgcgggagccgcagggccgccgccgagcgggccgcggcagggacggtctgcaaactaccagccctggcggggccgcgcgcggcgcgtccacactcagccccgagacgcagcagaggcgctcctgtgggagctcagtcgaccagggcgggagtccgtcctcaatttctggcaaccttcccctagccaacctcaccaacttctccccgcttctgggctcgcggctctagaaggcagaaa

SEQ ID NO: 8988 - RNA, 6619 nt, Homo sapiens
  source 1..6619: mol_type = other RNA
accttcttgtataagcactgtgctaaacactgaatcctcacaaaaccctaagtgctaagaaagctagggtaatttttttctgcattcaagactctacagctaatttggtcttttgctataaaaacttggtctcccactttttgttgaagcgaacaagaatcacaggaactcaccctcagcttcacgaaactcccagcttcctaaatgagcatgaatctatttatgtccatccgtctactcacatgaagatgctctgcagctccacagggatggatgggattagaataaagccaatatggaaattaaaatacttttaaataaataaaataatccaggcttgggatagtaacacatacaacagagcctgtcgttaacaaaatagacttttctttttaaatcaagaatttttggccagaggtgagggtggcaatgtctaatatacacaagctaggtaaaccaccttggagaaatggggtggccaccgtggtctgccctaaaaggcacacacctacctacagacatacagtttcagtccaacacatcatactgatgtcaaccctgtcagtgagctgcactgggctccactcccaaaggggaagctcattattcacttttattaaatcttgcattcactaaagaaacaaaaaaggggtgcacgttctttccctttcatgatgctaaagtatttcttctccaagcagggccctgaactccttggatgcacccattcacatgattctgcctcagccacacctcagcaagtgcgtgggtggcagggaacacaggctggttgacacgttggcaaccagcagtcccaaggtagacccaaaggtatggcagaatccagccctttcttgaggttctcaaggcttcacaccctcctctgtgggtggaagtgcacatgcatacacgctatggcctggcgggggggttatagggagcgtctggtgtccagcttcaacagctacagtggctcaagaacatgtcctgtctcttagctggaggagtctgctattgcccttcaacagcatccggattccaaaaaccccaaagaaaaacgaaaaggcacatcaaggaaacaaatatcactaaagaaactgactaatatctccaaacgcacagcaaacacacaaaaaagcaaactgtaatgagcagtgacacaaacccagtccaaacaaaaatgaaaagcatctccatttatacatgtgcaaatcaaactgcatacacaaaataaatgcggtgtttaccagcattcaaagaagtctttttactcctcaaagtatctacctttcaatggaaagctttctcttttagtaaattagatgaatgttttccctcaagttttttaagagcttaggatcacaatggggaaaataatccaaaaaaacaggcaagatattatagcggggaaaaacattaatcataacttaggatttctctccccatggaactgttatcagctataaatcggtttaggattctatcaagatcagcaatggcaaaacctccgcaggcttccagcccacacaggggcaccttcctctcctcttccatgcagggcagttggaagccccctccccagtttcctctccaggatcactgactagacctgggccaagtctgaggaggcctgggagccagtacacattcaggggtcactgactcttcagataatgccctaaacaactggagtgtgggcttgtttgctccaagagcagctgccctgtcagtggaactccggcgcacttccactcaatactggactgggggggatgaaagagggatttttaaatggcagaaaagtgttcttctgggctgtctggcccgggcagggcgggttgtgacttggaaaagaaggggaaggtagggaggccttgaacttagggacagccagcaaatgatccttgcagcttttggaacacaaggcagggctaaggttacctttcagcttccttgcttaagtagcagtggctaagtgggttaaactttgctcggcctgcaggctccccctgttggtcagatacttgcattgacatcctcagtgttcaatgctcctggaagagcccaggagagggcggcactggcccagggattgcaggtcagggaactctagcaaattcccacaccctagggtacagccaagaggcccattcacaaggaaaaagctcttccttacagcaaggatgccagtcatctgccctcctactgcaggaaactgcccttgcttaaaagaaatgcacaggctcatacacacacacacacacacacacacacacacacacacacacacacacactcactcaccaaggtttcctttggacttctgcccttcttcctaggcccaagcagaggctattctcagccaggtctggaggcgcccctgtgatgatgctcagggcagaggcctccccatggtactctacctggcagatgtgcttgggggccacctaaggagtggaggaggccccgggtgccccccaccctcctcttagactggagatacaattgagacgcactgagcagggatctcagtgggcctaagaaaaaaggctggctgcacatttgtgtagcaattgagaaagaagcagaatgtaacttcccagacttaaaggccccacactaactctagtccccatgaagcggaattcttcctttccctcacattctgaaagctaccagccattacgccttgcccatcagttctgcccagcggaggctccactgggccgccctctgttagcaggaagggtgcttggaagccccggcacagagcacatcattgagcgactgaggcgcccagcagaggccaagtggaggacgccaaccgctcacattaggcagaaggggtctcacttgcatcagcatggagatgtcaggggcttttcagaaacttacaaacttgtacagagcatggcagcaatgattcagtggggtgggaacttatacaaaggcagagcatgggggggtccagggtttggaaggtggggtccagtgtgtctgaccaggccaacctgatgactgattactcaacaagtcagagtgatcctgcctgaaggaaaagccagcaccagattcccacctttgcgagctacaccctcaggtgagtagccaggacagggcactgcattcatcctgagctgcccccactcccccagcagacatcaagagcccccttccctggactttggtgccatcagaggggacacaacacaagcccacctgtcaggagcccagctccggtcgcgccacaaattcttaaggaccgacttcactcctgtccaaatcttggctcaaagataatcctctccaagtccatgaacagcgtgagtctttcatctctactttcctcctcatagcggggctggagggagggtgagtttaccagaaactccaaaatccctcaatcctgtatttccttcccaaagggattctaaaagaaattacggccaaggtatgtgtctgggcatggggacatggaggaaaggggcctcatctcctttttcgtccctggctgggctctctggacaacacaggcacgtccccctgactgaggcagcccatgctctaggtgccatctatgacgatgccctggggagtttggctgtgcttccaaagcaaaagtttcttttgttctgctgccatctgttttgagctgccaggtccccatggctgtccctgagcaggccaccagccccacggcacacggtctctctcctgcaccctgcccaaagcagacagaacaacagtatagtgaaggtggatgattaacagtggaaataaaagaagcctgtgatcaatccctcctctccctcccgcggtcccctccctcccacccgaataaataagttaatgggtttaggaatattcccattcagagttctttcccatcagctcaattcctcctgttttgttttaaaggactcttgagactttcttttgccctggagcagctgcagtgacagtcttcccacagttgctccttgagaaacagaaatgatgttgtgccagggacaagccaggctcctggcctgacatacgctcttgttttgttttggtgaagactccactgggttgctcggagtgcagcaagggcaatgccaattcagaaccttctacgaaaaagttcaggctcttgccagagtccctgcatgacttctgtccctggccctgcctgacggggctggggccactgtcttccccagcagcatggtgcagggctgagcaggtagctgctataggcagtctttgcagagagccacctggcccttgatgaagtcccggcaggggcagaccctctggtgcctggggtgggcgcctgcacagctgaagagcaggaggtcaccttgaaacacacagtgcttattcttagggtcaaaggagggcaccaggatgtccttggccagctctgagctttggcaggtcaccttgtacttcagcatgtccttgtccttgttgaggtgctggaagaaagaaggctcgcagatgagctggctctcctggcacacctgcttgcaggactgcccgggctcagcaagcttgacctgtagggcgctgaggggtggccacatcacttgcccatggcagaagtcctgtttttcaatgaaagcattgattctctgtagcatcccctcgcacgtaaattcatatggcatgtatggctcaatcttctgatttaaaattgctttcactgcatcctctacttcctcctgattgttgaggtcaacagtccacacatgtggccgcccgatgaaaacttcagcgtaaggatgctgggatgtcagctctctcagagttggcttgccaatgaaaaagtctgtgtttttgctgcttttgggtgggttgaacttgggattcagaaaagcacatccatttgcgatagcttccaggggagctgggccctcgtaagggaacccaagtccaacaaacaacttggtttctcgaagaaggaactgcaggtcccgtccactgaggataccatggtttttcacgtaactgggaatattctttgtgctggagccataaacagttgcatgcacttccatgtatgtgtgaataatgtccaagtagatcttcttattcttccagaagctatccactttgccatacacaagggactggttctgccttttgatttcattaatgtggtggatatcactggagttcaggtgctgctcaaccacaaaccccagaaagctgttgtctggggtatgagggaacatggtataaaactgctgagggttcagattccattttccccaaggggtcttgtggcctttcgattgggcataatttgcatgattaaattcgggttcagtaccaaatgaatcaaggactcggagcatgcactggtaatgaacccaggatggtccaagagttttcttgaattgagcaagtcctacaatatcaatgtaaatgagctcaacaattctgtctcctacagttgggcagccagatcggtttcctacaaccttcttcatgatttccttgagctcagccagtgaagctgaaatcctaatgtcatggcccagtaagtacagagatgtaattaaatcactccattgaactaattcaccaagagggccaccactgaaagctgtctctgcaatcttaaatccagattccttggtcaggagtcccaggtgaacgaggactttcttccgctttctcttttcaaggttctgcttttctgccagggacttgattgcttggatccatgcgtcagccattcgccggatccgtagtctcatccaccggaattcttcatgctttttcatcatactgtagagaatattaaaatctgtacgaatttccgccaatgaattatgatcagcttcttcgtagggattttttgctctccaaggtaaatgaggacaccaattttcaacctcactgaggtaaataaaaaaagagcaggtggatccatccactccatagtctgcgtagcagggatctgaacgccacatgtctttcatccacttgatctttccctcacagtgagggtagccgtccataggaggcaatacacatttttcttgagctccgttaatgatatctgccacattaattttctcaagtgcaaccaagctgggaacagctgtagtggagttggttgagtttgttccggtgccattgacaacaagattgtccaccttcgactccaacttgccaatgcgctgcaaaatgttatctaataacacagcaagggttttcttcagatcataagctgtcatgactccagcgtatggcccatccaccacattcctgttttcttctgccagtgccttgatgtaccttttgctgaggtccaggatctgctcgcgcagcatggagctgctttcaggctgagttcgctgctggatggtaaagtgcagaagcatcataccccaaatgaagccaaaagtcaccaggaaaaagcccagcttctgagaggacaacttccacggagtgaagagagccattgctctctggcaacttcacctgtccttggctcttaacgcgtagaagatagacacaaattcatggtgtaggttgagtgtgagagtctgctggtctcactctggctcctgtgtcagctggttgcctttcctcacttccattctctaagtaaaatgtcaactct

SEQ ID NO: 8989 - RNA, 7093 nt, Homo sapiens
  source 1..7093: mol_type = other RNA
accttcttgtataagcactgtgctaaacactgaatcctcacaaaaccctaagtgctaagaaagctagggtaatttttttctgcattcaagactctacagctaatttggtcttttgctataaaaacttggtctcccactttttgttgaagcgaacaagaatcacaggaactcaccctcagcttcacgaaactcccagcttcctaaatgagcatgaatctatttatgtccatccgtctactcacatgaagatgctctgcagctccacagggatggatgggattagaataaagccaatatggaaattaaaatacttttaaataaataaaataatccaggcttgggatagtaacacatacaacagagcctgtcgttaacaaaatagacttttctttttaaatcaagaatttttggccagaggtgagggtggcaatgtctaatatacacaagctaggtaaaccaccttggagaaatggggtggccaccgtggtctgccctaaaaggcacacacctacctacagacatacagtttcagtccaacacatcatactgatgtcaaccctgtcagtgagctgcactgggctccactcccaaaggggaagctcattattcacttttattaaatcttgcattcactaaagaaacaaaaaaggggtgcacgttctttccctttcatgatgctaaagtatttcttctccaagcagggccctgaactccttggatgcacccattcacatgattctgcctcagccacacctcagcaagtgcgtgggtggcagggaacacaggctggttgacacgttggcaaccagcagtcccaaggtagacccaaaggtatggcagaatccagccctttcttgaggttctcaaggcttcacaccctcctctgtgggtggaagtgcacatgcatacacgctatggcctggcgggggggttatagggagcgtctggtgtccagcttcaacagctacagtggctcaagaacatgtcctgtctcttagctggaggagtctgctattgcccttcaacagcatccggattccaaaaaccccaaagaaaaacgaaaaggcacatcaaggaaacaaatatcactaaagaaactgactaatatctccaaacgcacagcaaacacacaaaaaagcaaactgtaatgagcagtgacacaaacccagtccaaacaaaaatgaaaagcatctccatttatacatgtgcaaatcaaactgcatacacaaaataaatgcggtgtttaccagcattcaaagaagtctttttactcctcaaagtatctacctttcaatggaaagctttctcttttagtaaattagatgaatgttttccctcaagttttttaagagcttaggatcacaatggggaaaataatccaaaaaaacaggcaagatattatagcggggaaaaacattaatcataacttaggatttctctccccatggaactgttatcagctataaatcggtttaggattctatcaagatcagcaatggcaaaacctccgcaggcttccagcccacacaggggcaccttcctctcctcttccatgcagggcagttggaagccccctccccagtttcctctccaggatcactgactagacctgggccaagtctgaggaggcctgggagccagtacacattcaggggtcactgactcttcagataatgccctaaacaactggagtgtgggcttgtttgctccaagagcagctgccctgtcagtggaactccggcgcacttccactcaatactggactgggggggatgaaagagggatttttaaatggcagaaaagtgttcttctgggctgtctggcccgggcagggcgggttgtgacttggaaaagaaggggaaggtagggaggccttgaacttagggacagccagcaaatgatccttgcagcttttggaacacaaggcagggctaaggttacctttcagcttccttgcttaagtagcagtggctaagtgggttaaactttgctcggcctgcaggctccccctgttggtcagatacttgcattgacatcctcagtgttcaatgctcctggaagagcccaggagagggcggcactggcccagggattgcaggtcagggaactctagcaaattcccacaccctagggtacagccaagaggcccattcacaaggaaaaagctcttccttacagcaaggatgccagtcatctgccctcctactgcaggaaactgcccttgcttaaaagaaatgcacaggctcatacacacacacacacacacacacacacacacacacacacacacacacactcactcaccaaggtttcctttggacttctgcccttcttcctaggcccaagcagaggctattctcagccaggtctggaggcgcccctgtgatgatgctcagggcagaggcctccccatggtactctacctggcagatgtgcttgggggccacctaaggagtggaggaggccccgggtgccccccaccctcctcttagactggagatacaattgagacgcactgagcagggatctcagtgggcctaagaaaaaaggctggctgcacatttgtgtagcaattgagaaagaagcagaatgtaacttcccagacttaaaggccccacactaactctagtccccatgaagcggaattcttcctttccctcacattctgaaagctaccagccattacgccttgcccatcagttctgcccagcggaggctccactgggccgccctctgttagcaggaagggtgcttggaagccccggcacagagcacatcattgagcgactgaggcgcccagcagaggccaagtggaggacgccaaccgctcacattaggcagaaggggtctcacttgcatcagcatggagatgtcaggggcttttcagaaacttacaaacttgtacagagcatggcagcaatgattcagtggggtgggaacttatacaaaggcagagcatgggggggtccagggtttggaaggtggggtccagtgtgtctgaccaggccaacctgatgactgattactcaacaagtcagagtgatcctgcctgaaggaaaagccagcaccagattcccacctttgcgagctacaccctcaggtgagtagccaggacagggcactgcattcatcctgagctgcccccactcccccagcagacatcaagagcccccttccctggactttggtgccatcagaggggacacaacacaagcccacctgtcaggagcccagctccggtcgcgccacaaattcttaaggaccgacttcactcctgtccaaatcttggctcaaagataatcctctccaagtccatgaacagcgtgagtctttcatctctactttcctcctcatagcggggctggagggagggtgagtttaccagaaactccaaaatccctcaatcctgtatttccttcccaaagggattctaaaagaaattacggccaaggtatgtgtctgggcatggggacatggaggaaaggggcctcatctcctttttcgtccctggctgggctctctggacaacacaggcacgtccccctgactgaggcagcccatgctctaggtgccatctatgacgatgccctggggagtttggctgtgcttccaaagcaaaagtttcttttgttctgctgccatctgttttgagctgccaggtccccatggctgtccctgagcaggccaccagccccacggcacacggtctctctcctgcaccctgcccaaagcagacagaacaacagtatagtgaaggtggatgattaacagtggaaataaaagaagcctgtgatcaatccctcctctccctcccgcggtcccctccctcccacccgaataaataagttaatgggtttaggaatattcccattcagagttctttcccatcagctcaattcctcctgttttgttttaaaggactcttgagactttcttttgccctggagcagctgcagtgacagtcttcccacagttgctccttgagaaacagaaatgatgttgtgccagggacaagccaggctcctggcctgacatacgctcttgttttgttttggtgaagactccactgggttgctcggagtgcagcaagggcaatgccaattcagaaccttctacgaaaaagttcaggctcttgccagagtccctgcatgacttctgtccctggccctgcctgacggggctggggccactgtcttccccagcagcatggtgcagggctgagcaggtagctgctataggcagtctttgcagagagccacctggcccttgatgaagtcccggcaggggcagaccctctggtgcctggggtgggcgcctgcacagctgaagagcaggaggtcaccttgaaacacacagtgcttattcttagggtcaaaggagggcaccaggatgtccttggccagctctgagctttggcaggtcaccttgtacttcagcatgtccttgtccttgttgaggtgctggaagaaagaaggctcgcagatgagctggctctcctggcacacctgcttgcaggactgcccgggctcagcaagcttgacctgtagggcgctgaggggtggccacatcacttgcccatggcagaagtcctgtttttcaatgaaagcattgattctctgtagcatcccctcgcacgtaaattcatatggcatgtatggctcaatcttctgatttaaaattgctttcactgcatcctctacttcctcctgattgttgaggtcaacagtccacacatgtggccgcccgatgaaaacttcagcgtaaggatgctgggatgtcagctctctcagagttggcttgccaatgaaaaagtctgtgtttttgctgcttttgggtgggttgaacttgggattcagaaaagcacatccatttgcgatagcttccaggggagctgggccctcgtaagggaacccaagtccaacaaacaacttggtttctcgaagaaggaactgcaggtcccgtccactgaggataccatggtttttcacgtaactgggaatattctttgtgctggagccataaacagttgcatgcacttccatgtatgtgtgaataatgtccaagtagatcttcttattcttccagaagctatccactttgccatacacaagggactggttctgccttttgatttcattaatgtggtggatatcactggagttcaggtgctgctcaaccacaaaccccagaaagctgttgtctggggtatgagggaacatggtataaaactgctgagggttcagattccattttccccaaggggtcttgtggcctttcgattgggcataatttgcatgattaaattcgggttcagtaccaaatgaatcaaggactcggagcatgcactggtaatgaacccaggatggtccaagagttttcttgaattgagcaagtcctacaatatcaatgtaaatgagctcaacaattctgtctcctacagttgggcagccagatcggtttcctacaaccttcttcatgatttccttgagctcagccagtgaagctgaaatcctaatgtcatggcccagtaagtacagagatgtaattaaatcactccattgaactaattcaccaagagggccaccactgaaagctgtctctgcaatcttaaatccagattccttggtcaggagtcccaggtgaacgaggactttcttccgctttctcttttcaaggttctgcttttctgccagggacttgattgcttggatccatgcgtcagccattcgccggatccgtagtctcatccaccggaattcttcatgctttttcatcatactgtagagaatattaaaatctgtacgaatttccgccaatgaattatgatcagcttcttcgtagggattttttgctctccaaggtaaatgaggacaccaattttcaacctcactgaggtaaataaaaaaagagcaggtggatccatccactccatagtctgcgtagcagggatctgaacgccacatgtctttcatccacttgatctttccctcacagtgagggtagccgtccataggaggcaatacacatttttcttgagctccgttaatgatatctgccacattaattttctcaagtgcaaccaagctgggaacagctgtagtggagttggttgagtttgttccggtgccattgacaacaagattgtccaccttcgactccaacttgccaatgcgctgcaaaatgttatctaataacacagcaagggttttcttcagatcataagctgtcatgactccagcgtatggcccatccaccacattcctgttttcttctgccagtgccttgatgtaccttttgctgaggtccaggatctgctcgcgcagcatggagctgctttcaggctgagttcgctgctggatggtaaagtgcagaagcatcataccccaaatgaagccaaaagtcaccaggaaaaagcccagcttctgagaggacaacttccacggagtgaagagagccattgctctctggcaacttcacctgtccttggctcttaacgcgtagaagatagacacaaattcatggtgtaggttgagtgtgagagtctgctggtctcactctggctcctgtgtcagctggttgcctttcctcacttccattctgatgcttcagtcaaaggattcttctttgcaagcggcccaaaagaaaatggtagcaggatcttgaagcaattagctttcagagccctggatcactgttggtctgcctcttactgttttcccattgcctccttgttgggcagcagcagcagccgggagcacccgccggccgccgtgcccacgcggcccgaggcgcgaggtcgcgacgccccgagcctgcggcgcggctacctgggctggatcgcgcccggggccgccgccgcgggagccgcagggccgccgccgagcgggccgcggcagggacggtctgcaaactaccagccctggcggggccgcgcgcggcgcgtccacactcagccccgagacgcagcagaggcgctcctgtgggagctcagtcgaccagggcgggagtccgtcctcaatttctggcaaccttcccctagccaacctcaccaacttctccccgcttctgggctcgcggctctagaaggcagaaa

SEQ ID NO: 8990 - RNA, 7252 nt, Homo sapiens
  source 1..7252: mol_type = other RNA
accttcttgtataagcactgtgctaaacactgaatcctcacaaaaccctaagtgctaagaaagctagggtaatttttttctgcattcaagactctacagctaatttggtcttttgctataaaaacttggtctcccactttttgttgaagcgaacaagaatcacaggaactcaccctcagcttcacgaaactcccagcttcctaaatgagcatgaatctatttatgtccatccgtctactcacatgaagatgctctgcagctccacagggatggatgggattagaataaagccaatatggaaattaaaatacttttaaataaataaaataatccaggcttgggatagtaacacatacaacagagcctgtcgttaacaaaatagacttttctttttaaatcaagaatttttggccagaggtgagggtggcaatgtctaatatacacaagctaggtaaaccaccttggagaaatggggtggccaccgtggtctgccctaaaaggcacacacctacctacagacatacagtttcagtccaacacatcatactgatgtcaaccctgtcagtgagctgcactgggctccactcccaaaggggaagctcattattcacttttattaaatcttgcattcactaaagaaacaaaaaaggggtgcacgttctttccctttcatgatgctaaagtatttcttctccaagcagggccctgaactccttggatgcacccattcacatgattctgcctcagccacacctcagcaagtgcgtgggtggcagggaacacaggctggttgacacgttggcaaccagcagtcccaaggtagacccaaaggtatggcagaatccagccctttcttgaggttctcaaggcttcacaccctcctctgtgggtggaagtgcacatgcatacacgctatggcctggcgggggggttatagggagcgtctggtgtccagcttcaacagctacagtggctcaagaacatgtcctgtctcttagctggaggagtctgctattgcccttcaacagcatccggattccaaaaaccccaaagaaaaacgaaaaggcacatcaaggaaacaaatatcactaaagaaactgactaatatctccaaacgcacagcaaacacacaaaaaagcaaactgtaatgagcagtgacacaaacccagtccaaacaaaaatgaaaagcatctccatttatacatgtgcaaatcaaactgcatacacaaaataaatgcggtgtttaccagcattcaaagaagtctttttactcctcaaagtatctacctttcaatggaaagctttctcttttagtaaattagatgaatgttttccctcaagttttttaagagcttaggatcacaatggggaaaataatccaaaaaaacaggcaagatattatagcggggaaaaacattaatcataacttaggatttctctccccatggaactgttatcagctataaatcggtttaggattctatcaagatcagcaatggcaaaacctccgcaggcttccagcccacacaggggcaccttcctctcctcttccatgcagggcagttggaagccccctccccagtttcctctccaggatcactgactagacctgggccaagtctgaggaggcctgggagccagtacacattcaggggtcactgactcttcagataatgccctaaacaactggagtgtgggcttgtttgctccaagagcagctgccctgtcagtggaactccggcgcacttccactcaatactggactgggggggatgaaagagggatttttaaatggcagaaaagtgttcttctgggctgtctggcccgggcagggcgggttgtgacttggaaaagaaggggaaggtagggaggccttgaacttagggacagccagcaaatgatccttgcagcttttggaacacaaggcagggctaaggttacctttcagcttccttgcttaagtagcagtggctaagtgggttaaactttgctcggcctgcaggctccccctgttggtcagatacttgcattgacatcctcagtgttcaatgctcctggaagagcccaggagagggcggcactggcccagggattgcaggtcagggaactctagcaaattcccacaccctagggtacagccaagaggcccattcacaaggaaaaagctcttccttacagcaaggatgccagtcatctgccctcctactgcaggaaactgcccttgcttaaaagaaatgcacaggctcatacacacacacacacacacacacacacacacacacacacacacacacactcactcaccaaggtttcctttggacttctgcccttcttcctaggcccaagcagaggctattctcagccaggtctggaggcgcccctgtgatgatgctcagggcagaggcctccccatggtactctacctggcagatgtgcttgggggccacctaaggagtggaggaggccccgggtgccccccaccctcctcttagactggagatacaattgagacgcactgagcagggatctcagtgggcctaagaaaaaaggctggctgcacatttgtgtagcaattgagaaagaagcagaatgtaacttcccagacttaaaggccccacactaactctagtccccatgaagcggaattcttcctttccctcacattctgaaagctaccagccattacgccttgcccatcagttctgcccagcggaggctccactgggccgccctctgttagcaggaagggtgcttggaagccccggcacagagcacatcattgagcgactgaggcgcccagcagaggccaagtggaggacgccaaccgctcacattaggcagaaggggtctcacttgcatcagcatggagatgtcaggggcttttcagaaacttacaaacttgtacagagcatggcagcaatgattcagtggggtgggaacttatacaaaggcagagcatgggggggtccagggtttggaaggtggggtccagtgtgtctgaccaggccaacctgatgactgattactcaacaagtcagagtgatcctgcctgaaggaaaagccagcaccagattcccacctttgcgagctacaccctcaggtgagtagccaggacagggcactgcattcatcctgagctgcccccactcccccagcagacatcaagagcccccttccctggactttggtgccatcagaggggacacaacacaagcccacctgtcaggagcccagctccggtcgcgccacaaattcttaaggaccgacttcactcctgtccaaatcttggctcaaagataatcctctccaagtccatgaacagcgtgagtctttcatctctactttcctcctcatagcggggctggagggagggtgagtttaccagaaactccaaaatccctcaatcctgtatttccttcccaaagggattctaaaagaaattacggccaaggtatgtgtctgggcatggggacatggaggaaaggggcctcatctcctttttcgtccctggctgggctctctggacaacacaggcacgtccccctgactgaggcagcccatgctctaggtgccatctatgacgatgccctggggagtttggctgtgcttccaaagcaaaagtttcttttgttctgctgccatctgttttgagctgccaggtccccatggctgtccctgagcaggccaccagccccacggcacacggtctctctcctgcaccctgcccaaagcagacagaacaacagtatagtgaaggtggatgattaacagtggaaataaaagaagcctgtgatcaatccctcctctccctcccgcggtcccctccctcccacccgaataaataagttaatgggtttaggaatattcccattcagagttctttcccatcagctcaattcctcctgttttgttttaaaggactcttgagactttcttttgccctggagcagctgcagtgacagtcttcccacagttgctccttgagaaacagaaatgatgttgtgccagggacaagccaggctcctggcctgacatacgctcttgttttgttttggtgaagactccactgggttgctcggagtgcagcaagggcaatgccaattcagaaccttctacgaaaaagttcaggctcttgccagagtccctgcatgacttctgtccctggccctgcctgacggggctggggccactgtcttccccagcagcatggtgcagggctgagcaggtagctgctataggcagtctttgcagagagccacctggcccttgatgaagtcccggcaggggcagaccctctggtgcctggggtgggcgcctgcacagctgaagagcaggaggtcaccttgaaacacacagtgcttattcttagggtcaaaggagggcaccaggatgtccttggccagctctgagctttggcaggtcaccttgtacttcagcatgtccttgtccttgttgaggtgctggaagaaagaaggctcgcagatgagctggctctcctggcacacctgcttgcaggactgcccgggctcagcaagcttgacctgtagggcgctgaggggtggccacatcacttgcccatggcagaagtcctgtttttcaatgaaagcattgattctctgtagcatcccctcgcacgtaaattcatatggcatgtatggctcaatcttctgatttaaaattgctttcactgcatcctctacttcctcctgattgttgaggtcaacagtccacacatgtggccgcccgatgaaaacttcagcgtaaggatgctgggatgtcagctctctcagagttggcttgccaatgaaaaagtctgtgtttttgctgcttttgggtgggttgaacttgggattcagaaaagcacatccatttgcgatagcttccaggggagctgggccctcgtaagggaacccaagtccaacaaacaacttggtttctcgaagaaggaactgcaggtcccgtccactgaggataccatggtttttcacgtaactgggaatattctttgtgctggagccataaacagttgcatgcacttccatgtatgtgtgaataatgtccaagtagatcttcttattcttccagaagctatccactttgccatacacaagggactggttctgccttttgatttcattaatgtggtggatatcactggagttcaggtgctgctcaaccacaaaccccagaaagctgttgtctggggtatgagggaacatggtataaaactgctgagggttcagattccattttccccaaggggtcttgtggcctttcgattgggcataatttgcatgattaaattcgggttcagtaccaaatgaatcaaggactcggagcatgcactggtaatgaacccaggatggtccaagagttttcttgaattgagcaagtcctacaatatcaatgtaaatgagctcaacaattctgtctcctacagttgggcagccagatcggtttcctacaaccttcttcatgatttccttgagctcagccagtgaagctgaaatcctaatgtcatggcccagtaagtacagagatgtaattaaatcactccattgaactaattcaccaagagggccaccactgaaagctgtctctgcaatcttaaatccagattccttggtcaggagtcccaggtgaacgaggactttcttccgctttctcttttcaaggttctgcttttctgccagggacttgattgcttggatccatgcgtcagccattcgccggatccgtagtctcatccaccggaattcttcatgctttttcatcatactgtagagaatattaaaatctgtacgaatttccgccaatgaattatgatcagcttcttcgtagggattttttgctctccaaggtaaatgaggacaccaattttcaacctcactgaggtaaataaaaaaagagcaggtggatccatccactccatagtctgcgtagcagggatctgaacgccacatgtctttcatccacttgatctttccctcacagtgagggtagccgtccataggaggcaatacacatttttcttgagctccgttaatgatatctgccacattaattttctcaagtgcaaccaagctgggaacagctgtagtggagttggttgagtttgttccggtgccattgacaacaagattgtccaccttcgactccaacttgccaatgcgctgcaaaatgttatctaataacacagcaagggttttcttcagatcataagctgtcatgactccagcgtatggcccatccaccacattcctgttttcttctgccagtgccttgatgtaccttttgctgaggtccaggatctgctcgcgcagcatggagctgctttcaggctgagttcgctgctggatggtaaagtgcagaagcatcataccccaaatgaagccaaaagtcaccaggaaaaagcccagcttctgagaggacaacttccacggagtgaagagagccattgctctctggcaacttcacctgtccttggctcttaacgcgtagaagatagacacaaattcatggtgtaggttgagtgtgagagtctgctggtctcactctggctcctgtgtcagctggttgcctttcctcacttccattctgatgcttcagtcaaaggattcttctttgcaagcggcccaaaagaaaatggtagcaggatcttgaagcaattagctttcagagccctggatcactgttggtctgcctcttactgttttcccattgccttgttccttcccactgacgcctcaacacaacaaaatcatcttcaacctttataaagatggttagagatctctggcaaagaaatgtgtcaattctcctgaaagaaagaaaaaaaaagcacatgaaaagatgctcaacatcattagtcattagaggaaatgcaaatcaaaaccacaatgagatactaacttcacactcataaggacatacagataagaacaagtgttggtgaagatgtggagaaattggaaccctcatctaccactggtgggaatatcaaatggcgcagccagtgtgggaaataatctggcagtacctcaaatagttaaacatggagttactgtatgatccaaacaattctgcttctaggaactctcccaagagaaatgaaaatacgtgtctacacaaaaacttgtacacagaagtactcagcagcagtatccatactcagcagcattatccataataaacaaaagtaaaaccagcctaatgtgcatcaactgaggaaatggaaacaaaactgccatat

SEQ ID NO: 8991 - RNA, 6957 nt, Homo sapiens
  source 1..6957: mol_type = other RNA
accttcttgtataagcactgtgctaaacactgaatcctcacaaaaccctaagtgctaagaaagctagggtaatttttttctgcattcaagactctacagctaatttggtcttttgctataaaaacttggtctcccactttttgttgaagcgaacaagaatcacaggaactcaccctcagcttcacgaaactcccagcttcctaaatgagcatgaatctatttatgtccatccgtctactcacatgaagatgctctgcagctccacagggatggatgggattagaataaagccaatatggaaattaaaatacttttaaataaataaaataatccaggcttgggatagtaacacatacaacagagcctgtcgttaacaaaatagacttttctttttaaatcaagaatttttggccagaggtgagggtggcaatgtctaatatacacaagctaggtaaaccaccttggagaaatggggtggccaccgtggtctgccctaaaaggcacacacctacctacagacatacagtttcagtccaacacatcatactgatgtcaaccctgtcagtgagctgcactgggctccactcccaaaggggaagctcattattcacttttattaaatcttgcattcactaaagaaacaaaaaaggggtgcacgttctttccctttcatgatgctaaagtatttcttctccaagcagggccctgaactccttggatgcacccattcacatgattctgcctcagccacacctcagcaagtgcgtgggtggcagggaacacaggctggttgacacgttggcaaccagcagtcccaaggtagacccaaaggtatggcagaatccagccctttcttgaggttctcaaggcttcacaccctcctctgtgggtggaagtgcacatgcatacacgctatggcctggcgggggggttatagggagcgtctggtgtccagcttcaacagctacagtggctcaagaacatgtcctgtctcttagctggaggagtctgctattgcccttcaacagcatccggattccaaaaaccccaaagaaaaacgaaaaggcacatcaaggaaacaaatatcactaaagaaactgactaatatctccaaacgcacagcaaacacacaaaaaagcaaactgtaatgagcagtgacacaaacccagtccaaacaaaaatgaaaagcatctccatttatacatgtgcaaatcaaactgcatacacaaaataaatgcggtgtttaccagcattcaaagaagtctttttactcctcaaagtatctacctttcaatggaaagctttctcttttagtaaattagatgaatgttttccctcaagttttttaagagcttaggatcacaatggggaaaataatccaaaaaaacaggcaagatattatagcggggaaaaacattaatcataacttaggatttctctccccatggaactgttatcagctataaatcggtttaggattctatcaagatcagcaatggcaaaacctccgcaggcttccagcccacacaggggcaccttcctctcctcttccatgcagggcagttggaagccccctccccagtttcctctccaggatcactgactagacctgggccaagtctgaggaggcctgggagccagtacacattcaggggtcactgactcttcagataatgccctaaacaactggagtgtgggcttgtttgctccaagagcagctgccctgtcagtggaactccggcgcacttccactcaatactggactgggggggatgaaagagggatttttaaatggcagaaaagtgttcttctgggctgtctggcccgggcagggcgggttgtgacttggaaaagaaggggaaggtagggaggccttgaacttagggacagccagcaaatgatccttgcagcttttggaacacaaggcagggctaaggttacctttcagcttccttgcttaagtagcagtggctaagtgggttaaactttgctcggcctgcaggctccccctgttggtcagatacttgcattgacatcctcagtgttcaatgctcctggaagagcccaggagagggcggcactggcccagggattgcaggtcagggaactctagcaaattcccacaccctagggtacagccaagaggcccattcacaaggaaaaagctcttccttacagcaaggatgccagtcatctgccctcctactgcaggaaactgcccttgcttaaaagaaatgcacaggctcatacacacacacacacacacacacacacacacacacacacacacacacactcactcaccaaggtttcctttggacttctgcccttcttcctaggcccaagcagaggctattctcagccaggtctggaggcgcccctgtgatgatgctcagggcagaggcctccccatggtactctacctggcagatgtgcttgggggccacctaaggagtggaggaggccccgggtgccccccaccctcctcttagactggagatacaattgagacgcactgagcagggatctcagtgggcctaagaaaaaaggctggctgcacatttgtgtagcaattgagaaagaagcagaatgtaacttcccagacttaaaggccccacactaactctagtccccatgaagcggaattcttcctttccctcacattctgaaagctaccagccattacgccttgcccatcagttctgcccagcggaggctccactgggccgccctctgttagcaggaagggtgcttggaagccccggcacagagcacatcattgagcgactgaggcgcccagcagaggccaagtggaggacgccaaccgctcacattaggcagaaggggtctcacttgcatcagcatggagatgtcaggggcttttcagaaacttacaaacttgtacagagcatggcagcaatgattcagtggggtgggaacttatacaaaggcagagcatgggggggtccagggtttggaaggtggggtccagtgtgtctgaccaggccaacctgatgactgattactcaacaagtcagagtgatcctgcctgaaggaaaagccagcaccagattcccacctttgcgagctacaccctcaggtgagtagccaggacagggcactgcattcatcctgagctgcccccactcccccagcagacatcaagagcccccttccctggactttggtgccatcagaggggacacaacacaagcccacctgtcaggagcccagctccggtcgcgccacaaattcttaaggaccgacttcactcctgtccaaatcttggctcaaagataatcctctccaagtccatgaacagcgtgagtctttcatctctactttcctcctcatagcggggctggagggagggtgagtttaccagaaactccaaaatccctcaatcctgtatttccttcccaaagggattctaaaagaaattacggccaaggtatgtgtctgggcatggggacatggaggaaaggggcctcatctcctttttcgtccctggctgggctctctggacaacacaggcacgtccccctgactgaggcagcccatgctctaggtgccatctatgacgatgccctggggagtttggctgtgcttccaaagcaaaagtttcttttgttctgctgccatctgttttgagctgccaggtccccatggctgtccctgagcaggccaccagccccacggcacacggtctctctcctgcaccctgcccaaagcagacagaacaacagtatagtgaaggtggatgattaacagtggaaataaaagaagcctgtgatcaatccctcctctccctcccgcggtcccctccctcccacccgaataaataagttaatgggtttaggaatattcccattcagagttctttcccatcagctcaattcctcctgttttgttttaaaggactcttgagactttcttttgccctggagcagctgcagtgacagtcttcccacagttgctccttgagaaacagaaatgatgttgtgccagggacaagccaggctcctggcctgacatacgctcttgttttgttttggtgaagactccactgggttgctcggagtgcagcaagggcaatgccaattcagaaccttctacgaaaaagttcaggctcttgccagagtccctgcatgacttctgtccctggccctgcctgacggggctggggccactgtcttccccagcagcatggtgcagggctgagcaggtagctgctataggcagtctttgcagagagccacctggcccttgatgaagtcccggcaggggcagaccctctggtgcctggggtgggcgcctgcacagctgaagagcaggaggtcaccttgaaacacacagtgcttattcttagggtcaaaggagggcaccaggatgtccttggccagctctgagctttggcaggtcaccttgtacttcagcatgtccttgtccttgttgaggtgctggaagaaagaaggctcgcagatgagctggctctcctggcacacctgcttgcaggactgcccgggctcagcaagcttgacctgtagggcgctgaggggtggccacatcacttgcccatggcagaagtcctgtttttcaatgaaagcattgattctctgtagcatcccctcgcacgtaaattcatatggcatgtatggctcaatcttctgatttaaaattgctttcactgcatcctctacttcctcctgattgttgaggtcaacagtccacacatgtggccgcccgatgaaaacttcagcgtaaggatgctgggatgtcagctctctcagagttggcttgccaatgaaaaagtctgtgtttttgctgcttttgggtgggttgaacttgggattcagaaaagcacatccatttgcgatagcttccaggggagctgggccctcgtaagggaacccaagtccaacaaacaacttggtttctcgaagaaggaactgcaggtcccgtccactgaggataccatggtttttcacgtaactgggaatattctttgtgctggagccataaacagttgcatgcacttccatgtatgtgtgaataatgtccaagtagatcttcttattcttccagaagctatccactttgccatacacaagggactggttctgccttttgatttcattaatgtggtggatatcactggagttcaggtgctgctcaaccacaaaccccagaaagctgttgtctggggtatgagggaacatggtataaaactgctgagggttcagattccattttccccaaggggtcttgtggcctttcgattgggcataatttgcatgattaaattcgggttcagtaccaaatgaatcaaggactcggagcatgcactggtaatgaacccaggatggtccaagagttttcttgaattgagcaagtcctacaatatcaatgtaaatgagctcaacaattctgtctcctacagttgggcagccagatcggtttcctacaaccttcttcatgatttccttgagctcagccagtgaagctgaaatcctaatgtcatggcccagtaagtacagagatgtaattaaatcactccattgaactaattcaccaagagggccaccactgaaagctgtctctgcaatcttaaatccagattccttggtcaggagtcccaggtgaacgaggactttcttccgctttctcttttcaaggttctgcttttctgccagggacttgattgcttggatccatgcgtcagccattcgccggatccgtagtctcatccaccggaattcttcatgctttttcatcatactgtagagaatattaaaatctgtacgaatttccgccaatgaattatgatcagcttcttcgtagggattttttgctctccaaggtaaatgaggacaccaattttcaacctcactgaggtaaataaaaaaagagcaggtggatccatccactccatagtctgcgtagcagggatctgaacgccacatgtctttcatccacttgatctttccctcacagtgagggtagccgtccataggaggcaatacacatttttcttgagctccgttaatgatatctgccacattaattttctcaagtgcaaccaagctgggaacagctgtagtggagttggttgagtttgttccggtgccattgacaacaagattgtccaccttcgactccaacttgccaatgcgctgcaaaatgttatctaataacacagcaagggttttcttcagatcataagctgtcatgactccagcgtatggcccatccaccacattcctgttttcttctgccagtgccttgatgtaccttttgctgaggtccaggatctgctcgcgcagcatggagctgctttcaggctgagttcgctgctggatggtaaagtgcagaagcatcataccccaaatgaagccaaaagtcaccaggaaaaagcccagcttctgagaggacaacttccacggagtgaagagagccattgctctctggcaacttcacctgtccttggctcttaacgcgtagaagatagacacaaattcatggtgtaggttgagtgtgagagtctgctggtctcactctggctcctgtgtcagctggttgcctttcctcacttccattctgctccttgttgggcagcagcagcagccgggagcacccgccggccgccgtgcccacgcggcccgaggcgcgaggtcgcgacgccccgagcctgcggcgcggctacctgggctggatcgcgcccggggccgccgccgcgggagccgcagggccgccgccgagcgggccgcggcagggacggtctgcaaactaccagccctggcggggccgcgcgcggcgcgtccacactcagccccgagacgcagcagaggcgctcctgtgggagctcagtcgaccagggcgggagtccgtcctcaatttctggcaaccttcccctagccaacctcaccaacttctccccgcttctgggctcgcggctct

SEQ ID NO: 8992 - RNA, 6790 nt, Homo sapiens
  source 1..6790: mol_type = other RNA
accttcttgtataagcactgtgctaaacactgaatcctcacaaaaccctaagtgctaagaaagctagggtaatttttttctgcattcaagactctacagctaatttggtcttttgctataaaaacttggtctcccactttttgttgaagcgaacaagaatcacaggaactcaccctcagcttcacgaaactcccagcttcctaaatgagcatgaatctatttatgtccatccgtctactcacatgaagatgctctgcagctccacagggatggatgggattagaataaagccaatatggaaattaaaatacttttaaataaataaaataatccaggcttgggatagtaacacatacaacagagcctgtcgttaacaaaatagacttttctttttaaatcaagaatttttggccagaggtgagggtggcaatgtctaatatacacaagctaggtaaaccaccttggagaaatggggtggccaccgtggtctgccctaaaaggcacacacctacctacagacatacagtttcagtccaacacatcatactgatgtcaaccctgtcagtgagctgcactgggctccactcccaaaggggaagctcattattcacttttattaaatcttgcattcactaaagaaacaaaaaaggggtgcacgttctttccctttcatgatgctaaagtatttcttctccaagcagggccctgaactccttggatgcacccattcacatgattctgcctcagccacacctcagcaagtgcgtgggtggcagggaacacaggctggttgacacgttggcaaccagcagtcccaaggtagacccaaaggtatggcagaatccagccctttcttgaggttctcaaggcttcacaccctcctctgtgggtggaagtgcacatgcatacacgctatggcctggcgggggggttatagggagcgtctggtgtccagcttcaacagctacagtggctcaagaacatgtcctgtctcttagctggaggagtctgctattgcccttcaacagcatccggattccaaaaaccccaaagaaaaacgaaaaggcacatcaaggaaacaaatatcactaaagaaactgactaatatctccaaacgcacagcaaacacacaaaaaagcaaactgtaatgagcagtgacacaaacccagtccaaacaaaaatgaaaagcatctccatttatacatgtgcaaatcaaactgcatacacaaaataaatgcggtgtttaccagcattcaaagaagtctttttactcctcaaagtatctacctttcaatggaaagctttctcttttagtaaattagatgaatgttttccctcaagttttttaagagcttaggatcacaatggggaaaataatccaaaaaaacaggcaagatattatagcggggaaaaacattaatcataacttaggatttctctccccatggaactgttatcagctataaatcggtttaggattctatcaagatcagcaatggcaaaacctccgcaggcttccagcccacacaggggcaccttcctctcctcttccatgcagggcagttggaagccccctccccagtttcctctccaggatcactgactagacctgggccaagtctgaggaggcctgggagccagtacacattcaggggtcactgactcttcagataatgccctaaacaactggagtgtgggcttgtttgctccaagagcagctgccctgtcagtggaactccggcgcacttccactcaatactggactgggggggatgaaagagggatttttaaatggcagaaaagtgttcttctgggctgtctggcccgggcagggcgggttgtgacttggaaaagaaggggaaggtagggaggccttgaacttagggacagccagcaaatgatccttgcagcttttggaacacaaggcagggctaaggttacctttcagcttccttgcttaagtagcagtggctaagtgggttaaactttgctcggcctgcaggctccccctgttggtcagatacttgcattgacatcctcagtgttcaatgctcctggaagagcccaggagagggcggcactggcccagggattgcaggtcagggaactctagcaaattcccacaccctagggtacagccaagaggcccattcacaaggaaaaagctcttccttacagcaaggatgccagtcatctgccctcctactgcaggaaactgcccttgcttaaaagaaatgcacaggctcatacacacacacacacacacacacacacacacacacacacacacacacactcactcaccaaggtttcctttggacttctgcccttcttcctaggcccaagcagaggctattctcagccaggtctggaggcgcccctgtgatgatgctcagggcagaggcctccccatggtactctacctggcagatgtgcttgggggccacctaaggagtggaggaggccccgggtgccccccaccctcctcttagactggagatacaattgagacgcactgagcagggatctcagtgggcctaagaaaaaaggctggctgcacatttgtgtagcaattgagaaagaagcagaatgtaacttcccagacttaaaggccccacactaactctagtccccatgaagcggaattcttcctttccctcacattctgaaagctaccagccattacgccttgcccatcagttctgcccagcggaggctccactgggccgccctctgttagcaggaagggtgcttggaagccccggcacagagcacatcattgagcgactgaggcgcccagcagaggccaagtggaggacgccaaccgctcacattaggcagaaggggtctcacttgcatcagcatggagatgtcaggggcttttcagaaacttacaaacttgtacagagcatggcagcaatgattcagtggggtgggaacttatacaaaggcagagcatgggggggtccagggtttggaaggtggggtccagtgtgtctgaccaggccaacctgatgactgattactcaacaagtcagagtgatcctgcctgaaggaaaagccagcaccagattcccacctttgcgagctacaccctcaggtgagtagccaggacagggcactgcattcatcctgagctgcccccactcccccagcagacatcaagagcccccttccctggactttggtgccatcagaggggacacaacacaagcccacctgtcaggagcccagctccggtcgcgccacaaattcttaaggaccgacttcactcctgtccaaatcttggctcaaagataatcctctccaagtccatgaacagcgtgagtctttcatctctactttcctcctcatagcggggctggagggagggtgagtttaccagaaactccaaaatccctcaatcctgtatttccttcccaaagggattctaaaagaaattacggccaaggtatgtgtctgggcatggggacatggaggaaaggggcctcatctcctttttcgtccctggctgggctctctggacaacacaggcacgtccccctgactgaggcagcccatgctctaggtgccatctatgacgatgccctggggagtttggctgtgcttccaaagcaaaagtttcttttgttctgctgccatctgttttgagctgccaggtccccatggctgtccctgagcaggccaccagccccacggcacacggtctctctcctgcaccctgcccaaagcagacagaacaacagtatagtgaaggtggatgattaacagtggaaataaaagaagcctgtgatcaatccctcctctccctcccgcggtcccctccctcccacccgaataaataagttaatgggtttaggaatattcccattcagagttctttcccatcagctcaattcctcctgttttgttttaaaggactcttgagactttcttttgccctggagcagctgcagtgacagtcttcccacagttgctccttgagaaacagaaatgatgttgtgccagggacaagccaggctcctggcctgacatacgctcttgttttgttttggtgaagactccactgggttgctcggagtgcagcaagggcaatgccaattcagaaccttctacgaaaaagttcaggctcttgccagagtccctgcatgacttctgtccctggccctgcctgacggggctggggccactgtcttccccagcagcatggtgcagggctgagcaggtagctgctataggcagtctttgcagagagccacctggcccttgatgaagtcccggcaggggcagaccctctggtgcctggggtgggcgcctgcacagctgaagagcaggaggtcaccttgaaacacacagtgcttattcttagggtcaaaggagggcaccaggatgtccttggccagctctgagctttggcaggtcaccttgtacttcagcatgtccttgtccttgttgaggtgctggaagaaagaaggctcgcagatgagctggctctcctggcacacctgcttgcaggactgcccgggctcagcaagcttgacctgtagggcgctgaggggtggccacatcacttgcccatggcagaagtcctgtttttcaatgaaagcattgattctctgtagcatcccctcgcacgtaaattcatatggcatgtatggctcaatcttctgatttaaaattgctttcactgcatcctctacttcctcctgattgttgaggtcaacagtccacacatgtggccgcccgatgaaaacttcagcgtaaggatgctgggatgtcagctctctcagagttggcttgccaatgaaaaagtctgtgtttttgctgcttttgggtgggttgaacttgggattcagaaaagcacatccatttgcgatagcttccaggggagctgggccctcgtaagggaacccaagtccaacaaacaacttggtttctcgaagaaggaactgcaggtcccgtccactgaggataccatggtttttcacgtaactgggaatattctttgtgctggagccataaacagttgcatgcacttccatgtatgtgtgaataatgtccaagtagatcttcttattcttccagaagctatccactttgccatacacaagggactggttctgccttttgatttcattaatgtggtggatatcactggagttcaggtgctgctcaaccacaaaccccagaaagctgttgtctggggtatgagggaacatggtataaaactgctgagggttcagattccattttccccaaggggtcttgtggcctttcgattgggcataatttgcatgattaaattcgggttcagtaccaaatgaatcaaggactcggagcatgcactggtaatgaacccaggatggtccaagagttttcttgaattgagcaagtcctacaatatcaatgtaaatgagctcaacaattctgtctcctacagttgggcagccagatcggtttcctacaaccttcttcatgatttccttgagctcagccagtgaagctgaaatcctaatgtcatggcccagtaagtacagagatgtaattaaatcactccattgaactaattcaccaagagggccaccactgaaagctgtctctgcaatcttaaatccagattccttggtcaggagtcccaggtgaacgaggactttcttccgctttctcttttcaaggttctgcttttctgccagggacttgattgcttggatccatgcgtcagccattcgccggatccgtagtctcatccaccggaattcttcatgctttttcatcatactgtagagaatattaaaatctgtacgaatttccgccaatgaattatgatcagcttcttcgtagggattttttgctctccaaggtaaatgaggacaccaattttcaacctcactgaggtaaataaaaaaagagcaggtggatccatccactccatagtctgcgtagcagggatctgaacgccacatgtctttcatccacttgatctttccctcacagtgagggtagccgtccataggaggcaatacacatttttcttgagctccgttaatgatatctgccacattaattttctcaagtgcaaccaagctgggaacagctgtagtggagttggttgagtttgttccggtgccattgacaacaagattgtccaccttcgactccaacttgccaatgcgctgcaaaatgttatctaataacacagcaagggttttcttcagatcataagctgtcatgactccagcgtatggcccatccaccacattcctgttttcttctgccagtgccttgatgtaccttttgctgaggtccaggatctgctcgcgcagcatggagctgctttcaggctgagttcgctgctggatggtaaagtgcagaagcatcataccccaaatgaagccaaaagtcaccaggaaaaagcccagcttctgagaggacaacttccacggagtgaagagagccattgctctctggcaacttcacctgtccttggctcttaacgcgtagaagatagacacaaattcatggtgtaggttgagtgtgagagtctgctggtctcactctggctcctgtgtcagctggttgcctttcctcacttccattctgctgtgaaggaggagaagaattagccaagtggtcatggcacaatacagcaaaataaaccagaagccatgttttcacttgaatacctctaagtaaaatgtcaactcttaaatttgctggttcaatatcttatgattcaggaactgtaagctgaggggaaatctggctaggcaacaagaagctaagcaattat

SEQ ID NO: 8993 - RNA, 6617 nt, Homo sapiens
  source 1..6617: mol_type = other RNA
accttcttgtataagcactgtgctaaacactgaatcctcacaaaaccctaagtgctaagaaagctagggtaatttttttctgcattcaagactctacagctaatttggtcttttgctataaaaacttggtctcccactttttgttgaagcgaacaagaatcacaggaactcaccctcagcttcacgaaactcccagcttcctaaatgagcatgaatctatttatgtccatccgtctactcacatgaagatgctctgcagctccacagggatggatgggattagaataaagccaatatggaaattaaaatacttttaaataaataaaataatccaggcttgggatagtaacacatacaacagagcctgtcgttaacaaaatagacttttctttttaaatcaagaatttttggccagaggtgagggtggcaatgtctaatatacacaagctaggtaaaccaccttggagaaatggggtggccaccgtggtctgccctaaaaggcacacacctacctacagacatacagtttcagtccaacacatcatactgatgtcaaccctgtcagtgagctgcactgggctccactcccaaaggggaagctcattattcacttttattaaatcttgcattcactaaagaaacaaaaaaggggtgcacgttctttccctttcatgatgctaaagtatttcttctccaagcagggccctgaactccttggatgcacccattcacatgattctgcctcagccacacctcagcaagtgcgtgggtggcagggaacacaggctggttgacacgttggcaaccagcagtcccaaggtagacccaaaggtatggcagaatccagccctttcttgaggttctcaaggcttcacaccctcctctgtgggtggaagtgcacatgcatacacgctatggcctggcgggggggttatagggagcgtctggtgtccagcttcaacagctacagtggctcaagaacatgtcctgtctcttagctggaggagtctgctattgcccttcaacagcatccggattccaaaaaccccaaagaaaaacgaaaaggcacatcaaggaaacaaatatcactaaagaaactgactaatatctccaaacgcacagcaaacacacaaaaaagcaaactgtaatgagcagtgacacaaacccagtccaaacaaaaatgaaaagcatctccatttatacatgtgcaaatcaaactgcatacacaaaataaatgcggtgtttaccagcattcaaagaagtctttttactcctcaaagtatctacctttcaatggaaagctttctcttttagtaaattagatgaatgttttccctcaagttttttaagagcttaggatcacaatggggaaaataatccaaaaaaacaggcaagatattatagcggggaaaaacattaatcataacttaggatttctctccccatggaactgttatcagctataaatcggtttaggattctatcaagatcagcaatggcaaaacctccgcaggcttccagcccacacaggggcaccttcctctcctcttccatgcagggcagttggaagccccctccccagtttcctctccaggatcactgactagacctgggccaagtctgaggaggcctgggagccagtacacattcaggggtcactgactcttcagataatgccctaaacaactggagtgtgggcttgtttgctccaagagcagctgccctgtcagtggaactccggcgcacttccactcaatactggactgggggggatgaaagagggatttttaaatggcagaaaagtgttcttctgggctgtctggcccgggcagggcgggttgtgacttggaaaagaaggggaaggtagggaggccttgaacttagggacagccagcaaatgatccttgcagcttttggaacacaaggcagggctaaggttacctttcagcttccttgcttaagtagcagtggctaagtgggttaaactttgctcggcctgcaggctccccctgttggtcagatacttgcattgacatcctcagtgttcaatgctcctggaagagcccaggagagggcggcactggcccagggattgcaggtcagggaactctagcaaattcccacaccctagggtacagccaagaggcccattcacaaggaaaaagctcttccttacagcaaggatgccagtcatctgccctcctactgcaggaaactgcccttgcttaaaagaaatgcacaggctcatacacacacacacacacacacacacacacacacacacacacacacacactcactcaccaaggtttcctttggacttctgcccttcttcctaggcccaagcagaggctattctcagccaggtctggaggcgcccctgtgatgatgctcagggcagaggcctccccatggtactctacctggcagatgtgcttgggggccacctaaggagtggaggaggccccgggtgccccccaccctcctcttagactggagatacaattgagacgcactgagcagggatctcagtgggcctaagaaaaaaggctggctgcacatttgtgtagcaattgagaaagaagcagaatgtaacttcccagacttaaaggccccacactaactctagtccccatgaagcggaattcttcctttccctcacattctgaaagctaccagccattacgccttgcccatcagttctgcccagcggaggctccactgggccgccctctgttagcaggaagggtgcttggaagccccggcacagagcacatcattgagcgactgaggcgcccagcagaggccaagtggaggacgccaaccgctcacattaggcagaaggggtctcacttgcatcagcatggagatgtcaggggcttttcagaaacttacaaacttgtacagagcatggcagcaatgattcagtggggtgggaacttatacaaaggcagagcatgggggggtccagggtttggaaggtggggtccagtgtgtctgaccaggccaacctgatgactgattactcaacaagtcagagtgatcctgcctgaaggaaaagccagcaccagattcccacctttgcgagctacaccctcaggtgagtagccaggacagggcactgcattcatcctgagctgcccccactcccccagcagacatcaagagcccccttccctggactttggtgccatcagaggggacacaacacaagcccacctgtcaggagcccagctccggtcgcgccacaaattcttaaggaccgacttcactcctgtccaaatcttggctcaaagataatcctctccaagtccatgaacagcgtgagtctttcatctctactttcctcctcatagcggggctggagggagggtgagtttaccagaaactccaaaatccctcaatcctgtatttccttcccaaagggattctaaaagaaattacggccaaggtatgtgtctgggcatggggacatggaggaaaggggcctcatctcctttttcgtccctggctgggctctctggacaacacaggcacgtccccctgactgaggcagcccatgctctaggtgccatctatgacgatgccctggggagtttggctgtgcttccaaagcaaaagtttcttttgttctgctgccatctgttttgagctgccaggtccccatggctgtccctgagcaggccaccagccccacggcacacggtctctctcctgcaccctgcccaaagcagacagaacaacagtatagtgaaggtggatgattaacagtggaaataaaagaagcctgtgatcaatccctcctctccctcccgcggtcccctccctcccacccgaataaataagttaatgggtttaggaatattcccattcagagttctttcccatcagctcaattcctcctgttttgttttaaaggactcttgagactttcttttgccctggagcagctgcagtgacagtcttcccacagttgctccttgagaaacagaaatgatgttgtgccagggacaagccaggctcctggcctgacatacgctcttgttttgttttggtgaagactccactgggttgctcggagtgcagcaagggcaatgccaattcagaaccttctacgaaaaagttcaggctcttgccagagtccctgcatgacttctgtccctggccctgcctgacggggctggggccactgtcttccccagcagcatggtgcagggctgagcaggtagctgctataggcagtctttgcagagagccacctggcccttgatgaagtcccggcaggggcagaccctctggtgcctggggtgggcgcctgcacagctgaagagcaggaggtcaccttgaaacacacagtgcttattcttagggtcaaaggagggcaccaggatgtccttggccagctctgagctttggcaggtcaccttgtacttcagcatgtccttgtccttgttgaggtgctggaagaaagaaggctcgcagatgagctggctctcctggcacacctgcttgcaggactgcccgggctcagcaagcttgacctgtagggcgctgaggggtggccacatcacttgcccatggcagaagtcctgtttttcaatgaaagcattgattctctgtagcatcccctcgcacgtaaattcatatggcatgtatggctcaatcttctgatttaaaattgctttcactgcatcctctacttcctcctgattgttgaggtcaacagtccacacatgtggccgcccgatgaaaacttcagcgtaaggatgctgggatgtcagctctctcagagttggcttgccaatgaaaaagtctgtgtttttgctgcttttgggtgggttgaacttgggattcagaaaagcacatccatttgcgatagcttccaggggagctgggccctcgtaagggaacccaagtccaacaaacaacttggtttctcgaagaaggaactgcaggtcccgtccactgaggataccatggtttttcacgtaactgggaatattctttgtgctggagccataaacagttgcatgcacttccatgtatgtgtgaataatgtccaagtagatcttcttattcttccagaagctatccactttgccatacacaagggactggttctgccttttgatttcattaatgtggtggatatcactggagttcaggtgctgctcaaccacaaaccccagaaagctgttgtctggggtatgagggaacatggtataaaactgctgagggttcagattccattttccccaaggggtcttgtggcctttcgattgggcataatttgcatgattaaattcgggttcagtaccaaatgaatcaaggactcggagcatgcactggtaatgaacccaggatggtccaagagttttcttgaattgagcaagtcctacaatatcaatgtaaatgagctcaacaattctgtctcctacagttgggcagccagatcggtttcctacaaccttcttcatgatttccttgagctcagccagtgaagctgaaatcctaatgtcatggcccagtaagtacagagatgtaattaaatcactccattgaactaattcaccaagagggccaccactgaaagctgtctctgcaatcttaaatccagattccttggtcaggagtcccaggtgaacgaggactttcttccgctttctcttttcaaggttctgcttttctgccagggacttgattgcttggatccatgcgtcagccattcgccggatccgtagtctcatccaccggaattcttcatgctttttcatcatactgtagagaatattaaaatctgtacgaatttccgccaatgaattatgatcagcttcttcgtagggattttttgctctccaaggtaaatgaggacaccaattttcaacctcactgaggtaaataaaaaaagagcaggtggatccatccactccatagtctgcgtagcagggatctgaacgccacatgtctttcatccacttgatctttccctcacagtgagggtagccgtccataggaggcaatacacatttttcttgagctccgttaatgatatctgccacattaattttctcaagtgcaaccaagctgggaacagctgtagtggagttggttgagtttgttccggtgccattgacaacaagattgtccaccttcgactccaacttgccaatgcgctgcaaaatgttatctaataacacagcaagggttttcttcagatcataagctgtcatgactccagcgtatggcccatccaccacattcctgttttcttctgccagtgccttgatgtaccttttgctgaggtccaggatctgctcgcgcagcatggagctgctttcaggctgagttcgctgctggatggtaaagtgcagaagcatcataccccaaatgaagccaaaagtcaccaggaaaaagcccagcttctgagaggacaacttccacggagtgaagagagccattgctctctggcaacttcacctgtccttggctcttaacgcgtagaagatagacacaaattcatggtgtaggttgagtgtgagagtctgctggtctcactctggctcctgtgtcagctggttgcctttcctcacttccattcttgttccttcccactgacg

SEQ ID NO: 8994 - RNA, 6929 nt, Homo sapiens
  source 1..6929: mol_type = other RNA
accttcttgtataagcactgtgctaaacactgaatcctcacaaaaccctaagtgctaagaaagctagggtaatttttttctgcattcaagactctacagctaatttggtcttttgctataaaaacttggtctcccactttttgttgaagcgaacaagaatcacaggaactcaccctcagcttcacgaaactcccagcttcctaaatgagcatgaatctatttatgtccatccgtctactcacatgaagatgctctgcagctccacagggatggatgggattagaataaagccaatatggaaattaaaatacttttaaataaataaaataatccaggcttgggatagtaacacatacaacagagcctgtcgttaacaaaatagacttttctttttaaatcaagaatttttggccagaggtgagggtggcaatgtctaatatacacaagctaggtaaaccaccttggagaaatggggtggccaccgtggtctgccctaaaaggcacacacctacctacagacatacagtttcagtccaacacatcatactgatgtcaaccctgtcagtgagctgcactgggctccactcccaaaggggaagctcattattcacttttattaaatcttgcattcactaaagaaacaaaaaaggggtgcacgttctttccctttcatgatgctaaagtatttcttctccaagcagggccctgaactccttggatgcacccattcacatgattctgcctcagccacacctcagcaagtgcgtgggtggcagggaacacaggctggttgacacgttggcaaccagcagtcccaaggtagacccaaaggtatggcagaatccagccctttcttgaggttctcaaggcttcacaccctcctctgtgggtggaagtgcacatgcatacacgctatggcctggcgggggggttatagggagcgtctggtgtccagcttcaacagctacagtggctcaagaacatgtcctgtctcttagctggaggagtctgctattgcccttcaacagcatccggattccaaaaaccccaaagaaaaacgaaaaggcacatcaaggaaacaaatatcactaaagaaactgactaatatctccaaacgcacagcaaacacacaaaaaagcaaactgtaatgagcagtgacacaaacccagtccaaacaaaaatgaaaagcatctccatttatacatgtgcaaatcaaactgcatacacaaaataaatgcggtgtttaccagcattcaaagaagtctttttactcctcaaagtatctacctttcaatggaaagctttctcttttagtaaattagatgaatgttttccctcaagttttttaagagcttaggatcacaatggggaaaataatccaaaaaaacaggcaagatattatagcggggaaaaacattaatcataacttaggatttctctccccatggaactgttatcagctataaatcggtttaggattctatcaagatcagcaatggcaaaacctccgcaggcttccagcccacacaggggcaccttcctctcctcttccatgcagggcagttggaagccccctccccagtttcctctccaggatcactgactagacctgggccaagtctgaggaggcctgggagccagtacacattcaggggtcactgactcttcagataatgccctaaacaactggagtgtgggcttgtttgctccaagagcagctgccctgtcagtggaactccggcgcacttccactcaatactggactgggggggatgaaagagggatttttaaatggcagaaaagtgttcttctgggctgtctggcccgggcagggcgggttgtgacttggaaaagaaggggaaggtagggaggccttgaacttagggacagccagcaaatgatccttgcagcttttggaacacaaggcagggctaaggttacctttcagcttccttgcttaagtagcagtggctaagtgggttaaactttgctcggcctgcaggctccccctgttggtcagatacttgcattgacatcctcagtgttcaatgctcctggaagagcccaggagagggcggcactggcccagggattgcaggtcagggaactctagcaaattcccacaccctagggtacagccaagaggcccattcacaaggaaaaagctcttccttacagcaaggatgccagtcatctgccctcctactgcaggaaactgcccttgcttaaaagaaatgcacaggctcatacacacacacacacacacacacacacacacacacacacacacacacactcactcaccaaggtttcctttggacttctgcccttcttcctaggcccaagcagaggctattctcagccaggtctggaggcgcccctgtgatgatgctcagggcagaggcctccccatggtactctacctggcagatgtgcttgggggccacctaaggagtggaggaggccccgggtgccccccaccctcctcttagactggagatacaattgagacgcactgagcagggatctcagtgggcctaagaaaaaaggctggctgcacatttgtgtagcaattgagaaagaagcagaatgtaacttcccagacttaaaggccccacactaactctagtccccatgaagcggaattcttcctttccctcacattctgaaagctaccagccattacgccttgcccatcagttctgcccagcggaggctccactgggccgccctctgttagcaggaagggtgcttggaagccccggcacagagcacatcattgagcgactgaggcgcccagcagaggccaagtggaggacgccaaccgctcacattaggcagaaggggtctcacttgcatcagcatggagatgtcaggggcttttcagaaacttacaaacttgtacagagcatggcagcaatgattcagtggggtgggaacttatacaaaggcagagcatgggggggtccagggtttggaaggtggggtccagtgtgtctgaccaggccaacctgatgactgattactcaacaagtcagagtgatcctgcctgaaggaaaagccagcaccagattcccacctttgcgagctacaccctcaggtgagtagccaggacagggcactgcattcatcctgagctgcccccactcccccagcagacatcaagagcccccttccctggactttggtgccatcagaggggacacaacacaagcccacctgtcaggagcccagctccggtcgcgccacaaattcttaaggaccgacttcactcctgtccaaatcttggctcaaagataatcctctccaagtccatgaacagcgtgagtctttcatctctactttcctcctcatagcggggctggagggagggtgagtttaccagaaactccaaaatccctcaatcctgtatttccttcccaaagggattctaaaagaaattacggccaaggtatgtgtctgggcatggggacatggaggaaaggggcctcatctcctttttcgtccctggctgggctctctggacaacacaggcacgtccccctgactgaggcagcccatgctctaggtgccatctatgacgatgccctggggagtttggctgtgcttccaaagcaaaagtttcttttgttctgctgccatctgttttgagctgccaggtccccatggctgtccctgagcaggccaccagccccacggcacacggtctctctcctgcaccctgcccaaagcagacagaacaacagtatagtgaaggtggatgattaacagtggaaataaaagaagcctgtgatcaatccctcctctccctcccgcggtcccctccctcccacccgaataaataagttaatgggtttaggaatattcccattcagagttctttcccatcagctcaattcctcctgttttgttttaaaggactcttgagactttcttttgccctggagcagctgcagtgacagtcttcccacagttgctccttgagaaacagaaatgatgttgtgccagggacaagccaggctcctggcctgacatacgctcttgttttgttttggtgaagactccactgggttgctcggagtgcagcaagggcaatgccaattcagaaccttctacgaaaaagttcaggctcttgccagagtccctgcatgacttctgtccctggccctgcctgacggggctggggccactgtcttccccagcagcatggtgcagggctgagcaggtagctgctataggcagtctttgcagagagccacctggcccttgatgaagtcccggcaggggcagaccctctggtgcctggggtgggcgcctgcacagctgaagagcaggaggtcaccttgaaacacacagtgcttattcttagggtcaaaggagggcaccaggatgtccttggccagctctgagctttggcaggtcaccttgtacttcagcatgtccttgtccttgttgaggtgctggaagaaagaaggctcgcagatgagctggctctcctggcacacctgcttgcaggactgcccgggctcagcaagcttgacctgtagggcgctgaggggtggccacatcacttgcccatggcagaagtcctgtttttcaatgaaagcattgattctctgtagcatcccctcgcacgtaaattcatatggcatgtatggctcaatcttctgatttaaaattgctttcactgcatcctctacttcctcctgattgttgaggtcaacagtccacacatgtggccgcccgatgaaaacttcagcgtaaggatgctgggatgtcagctctctcagagttggcttgccaatgaaaaagtctgtgtttttgctgcttttgggtgggttgaacttgggattcagaaaagcacatccatttgcgatagcttccaggggagctgggccctcgtaagggaacccaagtccaacaaacaacttggtttctcgaagaaggaactgcaggtcccgtccactgaggataccatggtttttcacgtaactgggaatattctttgtgctggagccataaacagttgcatgcacttccatgtatgtgtgaataatgtccaagtagatcttcttattcttccagaagctatccactttgccatacacaagggactggttctgccttttgatttcattaatgtggtggatatcactggagttcaggtgctgctcaaccacaaaccccagaaagctgttgtctggggtatgagggaacatggtataaaactgctgagggttcagattccattttccccaaggggtcttgtggcctttcgattgggcataatttgcatgattaaattcgggttcagtaccaaatgaatcaaggactcggagcatgcactggtaatgaacccaggatggtccaagagttttcttgaattgagcaagtcctacaatatcaatgtaaatgagctcaacaattctgtctcctacagttgggcagccagatcggtttcctacaaccttcttcatgatttccttgagctcagccagtgaagctgaaatcctaatgtcatggcccagtaagtacagagatgtaattaaatcactccattgaactaattcaccaagagggccaccactgaaagctgtctctgcaatcttaaatccagattccttggtcaggagtcccaggtgaacgaggactttcttccgctttctcttttcaaggttctgcttttctgccagggacttgattgcttggatccatgcgtcagccattcgccggatccgtagtctcatccaccggaattcttcatgctttttcatcatactgtagagaatattaaaatctgtacgaatttccgccaatgaattatgatcagcttcttcgtagggattttttgctctccaaggtaaatgaggacaccaattttcaacctcactgaggtaaataaaaaaagagcaggtggatccatccactccatagtctgcgtagcagggatctgaacgccacatgtctttcatccacttgatctttccctcacagtgagggtagccgtccataggaggcaatacacatttttcttgagctccgttaatgatatctgccacattaattttctcaagtgcaaccaagctgggaacagctgtagtggagttggttgagtttgttccggtgccattgacaacaagattgtccaccttcgactccaacttgccaatgcgctgcaaaatgttatctaataacacagcaagggttttcttcagatcataagctgtcatgactccagcgtatggcccatccaccacattcctgttttcttctgccagtgccttgatgtaccttttgctgaggtccaggatctgctcgcgcagcatggagctgctttcaggctgagttcgctgctggatggtaaagtgcagaagcatcataccccaaatgaagccaaaagtcaccaggaaaaagcccagcttctgagaggacaacttccacggagtgaagagagccattgctctctggcaacttcacctgtccttggctcttaacgcgtagaagatagacacaaattcatggtgtaggttgagtgtgagagtctgctggtctcactctggctcctgtgtcagctggttgcctttcctcacttccatttgaaatccgcactcttgtcatcttcctgggcacacagctggacctcgcttccctgccaggggtgaccaggtgactgtgttcttggcaatggaatgcgagtagaaagtgacgctaaccacagccagacccggccctaaaaacctccatgctggctcctccatcagatccccccaggcctgtgggctggaatgacagttacagcaggatgacctagagaacctgttttcaaaaagtcaaggcctaaagcctgggttgctacagaagttctttaaagaggtcattccctcccatcccatagaactgtttatcaacctaaaactatgaacaagaaa

SEQ ID NO: 8995 - RNA, 2941 nt, Homo sapiens
  source 1..2941: mol_type = other RNA
accttcttgtataagcactgtgctaaacacttacatcatctcatttaacctttacaagcacatacaattattcttctcactttacagatgggtaaagggatacataacttgtccaaggtcacatggcaaagctggaaatcaaatgaagttcagtcagatttcaattctgtgttacaaaacaccaaactaaagcatcttccatgtttatttttttctagatagttttgagcatccttaatgcctttaaattctccattgagttacgttagaatggttgtccttgtttcagtgaattagaaggctgaaatccagagagggcttgttcatctttgaggtaagatcaggacatttagttatggcatcaagtttgacagagagaaagccaaagctatggctctgcaaaccagctcggtcccttccttgagtataattttgtagtctagctctttttttttttttttttttcatagagatggggtctcgctaaattgcccaggttggtctcgaattcctggccctggcaatcctctcacctcagccttccaaagtgctcagattacagacatgagccactgtgcctagcttagctcttttttttttttttttttttgagatggagtcttgcactgtcacccaggctggagtgcagtggcacgatctcagctcactgcaacctccacctcccaggttcaagtgattctccttgcctcagcctcccaagtagctgggattacaggcgcccgccaccgtgcccggataattttttgtatttttagtagagacagggtttcactatgttggccaggctgatcttgaactcctgaccttgtgatccacccgcctcggcctcccaaagtgctgggattacaggcatgagccaccacgcccggccatctagattagttctttacattgaaagtaacatccagggtcactgatattctgagaaaattagaaccacctttgagttaagacttctagaaagacacatacgttgttatattttaattggaatcagacatttaatggcataaaaacattgcatatatggctttgctgttccgaatgtcatgaacttaaaatccaaatatgacataagcagttttaagacttattttggccagcctccccaatcccaaaggagatttaaaagtaataatgtaaaaaagttaaggtcaaggtgttttaaaatcaacatctcagctaatgactaaccctttgtttcctggggacttctgctctactgtgaaaactgctgagcttaacccgctgttgaacaactggttagttattagttccctgggtgattgtccctgaagttaagccatgctctggggacacatgaggcactttaattggggtagttactttttccaggttgggtacaatgtttggctctcaaaagcaaggtaaacagtttacagtcaaaaggaatgctctgtgattgtgtgcctttgggatcaagggttgagatcttagagtattctcataaacatctgtaccaggtgctcaaagatgtttgagggttgtcaagcaagctgttcaacttctgcattttctgtggatatgggcacaatgacccactcagatttttctcctagtgtcctgaatgacagctcatctacacagagtgaaactccagatatgtgacaagcagcatgggacagatgctgacaatcagaacagatgctggatgtaaacaactggtaaggctgcactggtgcatgctggcagaatcacctgctatgcatccagggagcaaatgcatctgcatgctcagcatgacaccagcttacctccctgtgcaaatcccctcccctaatcagtctcatccaaatcttctcctgcagtagcagcttctaaagctgcaagggcctccgccaccgctgcatcctcgtccacaatctccccatccccatctccatcggagccatgggtatcctcctgcctgtttcctgagtcaaccacaggcatggcatgaacaggacccttctcattaaagcagatgcttagaacttctgtttccacatcctcattcaatgaatcccagcttctcctcacagagaagggcgtattcaaaccatgctcccccactgggggctgaattccctctagggattcatcctcagtatggttcttgaaaacacagtccttttcattatgatcaacgttgtctccagctgggccccaatgctgaaggtaatctggggctggtatctggaagacatggtcttgtacttccaaggcaaaactttctgcctcagaaggagctctggagtctccatttctcatgacttgggtcccttctgaggccagcagcacacagtcctgtttcctggtgccccctccttccaggaagggttgagttgggggaacagtatttgcagtactggcccaggagcccctgtcatcctgggtggggctggaattcccagtgggctgtggagtggcagcagggccgatgccgttgacaccgcaggcatggtgttcccctccagcgtccccctgtgggagcggcccttggtgaggccagcagggctcccatggatcagctgtcctgctgctgctctcagtcttctttgagccctgcctctgagggtcatttttctgcaccaagacttcactgctccatttgccttttaatttatcagtgtcgtcttcatctagcttgcagctgttgacttcattgacatagccaggagagggcacttgaactggatcaaagagatagctttgtattattttacagcacctgcaccccatctggattgttttctgttaccacctgagggtcatgcttccgcgcctctccggagcttggcggggacagcctcttcctggttagaggttctgtcctctctcacctcgccctgagttttccttccccagcaacattccttctctagatcagacggacaggctctaatgtccaaggttgtgt

SEQ ID NO: 8996 - RNA, 3010 nt, Homo sapiens
  source 1..3010: mol_type = other RNA
accttcttgtataagcactgtgctaaacacttacatcatctcatttaacctttacaagcacatacaattattcttctcactttacagatgggtaaagggatacataacttgtccaaggtcacatggcaaagctggaaatcaaatgaagttcagtcagatttcaattctgtgttacaaaacaccaaactaaagcatcttccatgtttatttttttctagatagttttgagcatccttaatgcctttaaattctccattgagttacgttagaatggttgtccttgtttcagtgaattagaaggctgaaatccagagagggcttgttcatctttgaggtaagatcaggacatttagttatggcatcaagtttgacagagagaaagccaaagctatggctctgcaaaccagctcggtcccttccttgagtataattttgtagtctagctctttttttttttttttttttcatagagatggggtctcgctaaattgcccaggttggtctcgaattcctggccctggcaatcctctcacctcagccttccaaagtgctcagattacagacatgagccactgtgcctagcttagctcttttttttttttttttttttgagatggagtcttgcactgtcacccaggctggagtgcagtggcacgatctcagctcactgcaacctccacctcccaggttcaagtgattctccttgcctcagcctcccaagtagctgggattacaggcgcccgccaccgtgcccggataattttttgtatttttagtagagacagggtttcactatgttggccaggctgatcttgaactcctgaccttgtgatccacccgcctcggcctcccaaagtgctgggattacaggcatgagccaccacgcccggccatctagattagttctttacattgaaagtaacatccagggtcactgatattctgagaaaattagaaccacctttgagttaagacttctagaaagacacatacgttgttatattttaattggaatcagacatttaatggcataaaaacattgcatatatggctttgctgttccgaatgtcatgaacttaaaatccaaatatgacataagcagttttaagacttattttggccagcctccccaatcccaaaggagatttaaaagtaataatgtaaaaaagttaaggtcaaggtgttttaaaatcaacatctcagctaatgactaaccctttgtttcctggggacttctgctctactgtgaaaactgctgagcttaacccgctgttgaacaactggttagttattagttccctgggtgattgtccctgaagttaagccatgctctggggacacatgaggcactttaattggggtagttactttttccaggttgggtacaatgtttggctctcaaaagcaaggtaaacagtttacagtcaaaaggaatgctctgtgattgtgtgcctttgggatcaagggttgagatcttagagtattctcataaacatctgtaccaggtgctcaaagatgtttgagggttgtcaagcaagctgttcaacttctgcattttctgtggatatgggcacaatgacccactcagatttttctcctagtgtcctgaatgacagctcatctacacagagtgaaactccagatatgtgacaagcagcatgggacagatgctgacaatcagaacagatgctggatgtaaacaactggtaaggctgcactggtgcatgctggcagaatcacctgctatgcatccagggagcaaatgcatctgcatgctcagcatgacaccagcttacctccctgtgcaaatcccctcccctaatcagtctcatccaaatcttctcctgcagtagcagcttctaaagctgcaagggcctccgccaccgctgcatcctcgtccacaatctccccatccccatctccatcggagccatgggtatcctcctgcctgtttcctgagtcaaccacaggcatggcatgaacaggacccttctcattaaagcagatgcttagaacttctgtttccacatcctcattcaatgaatcccagcttctcctcacagagaagggcgtattcaaaccatgctcccccactgggggctgaattccctctagggattcatcctcagtatggttcttgaaaacacagtccttttcattatgatcaacgttgtctccagctgggccccaatgctgaaggtaatctggggctggtatctggaagacatggtcttgtacttccaaggcaaaactttctgcctcagaaggagctctggagtctccatttctcatgacttgggtcccttctgaggccagcagcacacagtcctgtttcctggtgccccctccttccaggaagggttgagttgggggaacagtatttgcagtactggcccaggagcccctgtcatcctgggtggggctggaattcccagtgggctgtggagtggcagcagggccgatgccgttgacaccgcaggcatggtgttcccctccagcgtccccctgtgggagcggcccttggtgaggccagcagggctcccatggatcagctgtcctgctgctgctctcagtcttctttgagccctgcctctgagggtcatttttctgcaccaagacttcactgctccatttgccttttaatttatcagtgtcgtcttcatctagcttgcagctgttgacttcattgacatagccaggagagggcacttgaactggatcaaagagatagctttgtattattttacagcacctgcaccccatctggattgttttctgttaccacctgttgtggatattgtctgttaggtttctctagaagtttaacttctcttcagttaatgcaatgcatattgaagtgctggggtgaaatgaactgatgtttgcaacttgctctggggccagacggcggcggcggcggcggcggcggggtcccggcgcccatggcttcgccggcctcgggcagccgcgccgggagacgctagcggctccgcgctgccctgagcccgcc

SEQ ID NO: 8997 - RNA, 3212 nt, Homo sapiens
  source 1..3212: mol_type = other RNA
accttcttgtataagcactgtgctaaacacttacatcatctcatttaacctttacaagcacatacaattattcttctcactttacagatgggtaaagggatacataacttgtccaaggtcacatggcaaagctggaaatcaaatgaagttcagtcagatttcaattctgtgttacaaaacaccaaactaaagcatcttccatgtttatttttttctagatagttttgagcatccttaatgcctttaaattctccattgagttacgttagaatggttgtccttgtttcagtgaattagaaggctgaaatccagagagggcttgttcatctttgaggtaagatcaggacatttagttatggcatcaagtttgacagagagaaagccaaagctatggctctgcaaaccagctcggtcccttccttgagtataattttgtagtctagctctttttttttttttttttttcatagagatggggtctcgctaaattgcccaggttggtctcgaattcctggccctggcaatcctctcacctcagccttccaaagtgctcagattacagacatgagccactgtgcctagcttagctcttttttttttttttttttttgagatggagtcttgcactgtcacccaggctggagtgcagtggcacgatctcagctcactgcaacctccacctcccaggttcaagtgattctccttgcctcagcctcccaagtagctgggattacaggcgcccgccaccgtgcccggataattttttgtatttttagtagagacagggtttcactatgttggccaggctgatcttgaactcctgaccttgtgatccacccgcctcggcctcccaaagtgctgggattacaggcatgagccaccacgcccggccatctagattagttctttacattgaaagtaacatccagggtcactgatattctgagaaaattagaaccacctttgagttaagacttctagaaagacacatacgttgttatattttaattggaatcagacatttaatggcataaaaacattgcatatatggctttgctgttccgaatgtcatgaacttaaaatccaaatatgacataagcagttttaagacttattttggccagcctccccaatcccaaaggagatttaaaagtaataatgtaaaaaagttaaggtcaaggtgttttaaaatcaacatctcagctaatgactaaccctttgtttcctggggacttctgctctactgtgaaaactgctgagcttaacccgctgttgaacaactggttagttattagttccctgggtgattgtccctgaagttaagccatgctctggggacacatgaggcactttaattggggtagttactttttccaggttgggtacaatgtttggctctcaaaagcaaggtaaacagtttacagtcaaaaggaatgctctgtgattgtgtgcctttgggatcaagggttgagatcttagagtattctcataaacatctgtaccaggtgctcaaagatgtttgagggttgtcaagcaagctgttcaacttctgcattttctgtggatatgggcacaatgacccactcagatttttctcctagtgtcctgaatgacagctcatctacacagagtgaaactccagatatgtgacaagcagcatgggacagatgctgacaatcagaacagatgctggatgtaaacaactggtaaggctgcactggtgcatgctggcagaatcacctgctatgcatccagggagcaaatgcatctgcatgctcagcatgacaccagcttacctccctgtgcaaatcccctcccctaatcagtctcatccaaatcttctcctgcagtagcagcttctaaagctgcaagggcctccgccaccgctgcatcctcgtccacaatctccccatccccatctccatcggagccatgggtatcctcctgcctgtttcctgagtcaaccacaggcatggcatgaacaggacccttctcattaaagcagatgcttagaacttctgtttccacatcctcattcaatgaatcccagcttctcctcacagagaagggcgtattcaaaccatgctcccccactgggggctgaattccctctagggattcatcctcagtatggttcttgaaaacacagtccttttcattatgatcaacgttgtctccagctgggccccaatgctgaaggtaatctggggctggtatctggaagacatggtcttgtacttccaaggcaaaactttctgcctcagaaggagctctggagtctccatttctcatgacttgggtcccttctgaggccagcagcacacagtcctgtttcctggtgccccctccttccaggaagggttgagttgggggaacagtatttgcagtactggcccaggagcccctgtcatcctgggtggggctggaattcccagtgggctgtggagtggcagcagggccgatgccgttgacaccgcaggcatggtgttcccctccagcgtccccctgtgggagcggcccttggtgaggccagcagggctcccatggatcagctgtcctgctgctgctctcagtcttctttgagccctgcctctgagggtcatttttctgcaccaagacttcactgctccatttgccttttaatttatcagtgtcgtcttcatctagcttgcagctgttgacttcattgacatagccaggagagggcacttgaactggatcaaagagatagctttgtattattttacagcacctgcaccccatctggattgttttctgttaccacctgttgtggatattgtctgttaggtttctctagaagtttaacttctcttcctgcacgccccgaggatgcggcggggctagggctcgaaaccctggagtacgatgtccgacatccccggggccggggtggcagtcccgggcgcactgaagcagaaaatccacgcgcttgttggcctctgagcacaaacgaccgcgccaaccgcctgccatcacgggaaactccggggtgcttactccaatgttgcgctggagagaagggagcttcctatgatcaagggactggagtacggggatacacaaaacaaatgcacccgctggcaaatagttgtgtactcccaaaccccgagaacttggcatttttcagtttcctccttatttctggcattcgccgcctagacctgctgtgagttccatggccagccctgtat

SEQ ID NO: 8998 - RNA, 2951 nt, Homo sapiens
  source 1..2951: mol_type = other RNA
accttcttgtataagcactgtgctaaacacttacatcatctcatttaacctttacaagcacatacaattattcttctcactttacagatgggtaaagggatacataacttgtccaaggtcacatggcaaagctggaaatcaaatgaagttcagtcagatttcaattctgtgttacaaaacaccaaactaaagcatcttccatgtttatttttttctagatagttttgagcatccttaatgcctttaaattctccattgagttacgttagaatggttgtccttgtttcagtgaattagaaggctgaaatccagagagggcttgttcatctttgaggtaagatcaggacatttagttatggcatcaagtttgacagagagaaagccaaagctatggctctgcaaaccagctcggtcccttccttgagtataattttgtagtctagctctttttttttttttttttttcatagagatggggtctcgctaaattgcccaggttggtctcgaattcctggccctggcaatcctctcacctcagccttccaaagtgctcagattacagacatgagccactgtgcctagcttagctcttttttttttttttttttttgagatggagtcttgcactgtcacccaggctggagtgcagtggcacgatctcagctcactgcaacctccacctcccaggttcaagtgattctccttgcctcagcctcccaagtagctgggattacaggcgcccgccaccgtgcccggataattttttgtatttttagtagagacagggtttcactatgttggccaggctgatcttgaactcctgaccttgtgatccacccgcctcggcctcccaaagtgctgggattacaggcatgagccaccacgcccggccatctagattagttctttacattgaaagtaacatccagggtcactgatattctgagaaaattagaaccacctttgagttaagacttctagaaagacacatacgttgttatattttaattggaatcagacatttaatggcataaaaacattgcatatatggctttgctgttccgaatgtcatgaacttaaaatccaaatatgacataagcagttttaagacttattttggccagcctccccaatcccaaaggagatttaaaagtaataatgtaaaaaagttaaggtcaaggtgttttaaaatcaacatctcagctaatgactaaccctttgtttcctggggacttctgctctactgtgaaaactgctgagcttaacccgctgttgaacaactggttagttattagttccctgggtgattgtccctgaagttaagccatgctctggggacacatgaggcactttaattggggtagttactttttccaggttgggtacaatgtttggctctcaaaagcaaggtaaacagtttacagtcaaaaggaatgctctgtgattgtgtgcctttgggatcaagggttgagatcttagagtattctcataaacatctgtaccaggtgctcaaagatgtttgagggttgtcaagcaagctgttcaacttctgcattttctgtggatatgggcacaatgacccactcagatttttctcctagtgtcctgaatgacagctcatctacacagagtgaaactccagatatgtgacaagcagcatgggacagatgctgacaatcagaacagatgctggatgtaaacaactggtaaggctgcactggtgcatgctggcagaatcacctgctatgcatccagggagcaaatgcatctgcatgctcagcatgacaccagcttacctccctgtgcaaatcccctcccctaatcagtctcatccaaatcttctcctgcagtagcagcttctaaagctgcaagggcctccgccaccgctgcatcctcgtccacaatctccccatccccatctccatcggagccatgggtatcctcctgcctgtttcctgagtcaaccacaggcatggcatgaacaggacccttctcattaaagcagatgcttagaacttctgtttccacatcctcattcaatgaatcccagcttctcctcacagagaagggcgtattcaaaccatgctcccccactgggggctgaattccctctagggattcatcctcagtatggttcttgaaaacacagtccttttcattatgatcaacgttgtctccagctgggccccaatgctgaaggtaatctggggctggtatctggaagacatggtcttgtacttccaaggcaaaactttctgcctcagaaggagctctggagtctccatttctcatgacttgggtcccttctgaggccagcagcacacagtcctgtttcctggtgccccctccttccaggaagggttgagttgggggaacagtatttgcagtactggcccaggagcccctgtcatcctgggtggggctggaattcccagtgggctgtggagtggcagcagggccgatgccgttgacaccgcaggcatggtgttcccctccagcgtccccctgtgggagcggcccttggtgaggccagcagggctcccatggatcagctgtcctgctgctgctctcagtcttctttgagccctgcctctgagggtcatttttctgcaccaagacttcactgctccatttgccttttaatttatcagtgtcgtcttcatctagcttgcagctgttgacttcattgacatagccaggagagggcacttgaactggatcaaagagatagctttgtattattttacagcacctgcaccccatctggattgttttctgttaccacctgttgtggatattgtctgttaggtttctctagaagtttaacttctcttcctggggccagacggcggcggcggcggcggcggcggggtcccggcgcccatggcttcgccggcctcgggcagccgcgccgggagacgctagcggctccgcgctgccctgagcccgcc

SEQ ID NO: 8999 - RNA, 6985 nt, Homo sapiens
  source 1..6985: mol_type = other RNA
accttcttgtataagcactgtgctaaacctggtaggtctggtggaggcagcggggttgtgtaagattgaaatgggggtggggtaaactgatgttaaactacataatttctactttggttcatggaattattcacataacctaaaaaatgtttttaaaaccaaatgtcaaatatcatttttttcccatgcatattgtaaacattgctttgcctttcttttctctctcatctctcaggcctttgtttggaaagagagaaataggtagtgcggctgattgtaatagcttgtttttattcacaagctttgcccagttcttctcaaagcacccctggtataaatatagctttataggatgtccgctaactccttcacttgctgctccgccctcaacgcaatgtatgactttgaggatgtattacatctttctaggtgtgaatgtctccatctgtcacctaaggataataatactgactaataaataaagcacttagagagtctcatgaaagatacaaagtcatattatatgctcaaaaagcctatggctcatggtccctttgccctatagatatttatgaaattgtattctcttaatcgcctcttacactttattagtttgatccttgtgagacatcttctaccttgtggtactgaaaagattgggtgcagcaaagagaagaacagtgacacctctgggaagcttatattttattactctaaagaacactgaagcaataattgacaatccagacctagcatatgagagtggttcaaaaaattttttaaaatctgatagatcaagatacagtagcctttatcccttgctccttctccttcctcaatgaacaattaaatgcatttggaccaaaaggtgataatttaaaatgaaggtataagcctgcctaaaatgatggttgtaaaattttattcttagtctcagaacactttctttaatcaaatatttgaggcctagttttggtaaaagggttcaatagtgttgcaggggatgattatagagccctctgtgaaatatttttgcatacattcctgatctggaattaaactagtggtctctgaacttcactgatctacctatctcagtaaaacatttttgcacacgccctcacatgtacatgatacaacagacacaaaaatggaactgtgaaaaagtaagataaaggtgaagtagcccatatttttacataattttctaaaattaatagcacaaagatattttccttcactaaaagttaggttattgacagtattctaatttttttttcagttttaaaatgacttgctggtggtgatgcatccaaacattattagctaatagactgtgtaattttatattcttagcacagagttcaactttaacttcactagtgctaagccggtctagaaatgtctgtccccagaaagatgtaaggatctggtgtgagggagaaggaatcggtgtaatattttatacagatcacacttagcattaaaatgagctaattaaaatgagcattacaatgttttggtcaacagtcttgagggcctatgaatttgcaatttccaatatgtactgtccttaattctacgcaacttctagaaaatttttttaaaatttccttgtttccatctcataactgaagaatggggaagcatcagttcttctgttctccaactgtttgtacatgtttgtattatcatgactacttcaatttgagatttcattttaagaatatttttaattctcttgttcattttgtgaaatacacaatataatctacgcattcacctacctgggcacagtgatatgtcttcatataccaaagacaaactcacaaataagagttatgcctgtagcctttctgagttttgaaattgctaccccatgttccatgtatggcatatgatcatctaacatatagagtatgtaggcaccagtgtctattcatataaagtgattgatgattataagatacaaaggacaaatataaattcttatatgttccttttgtgctcaatggattatgccactactatgctggtcttggccttcaagactgttgaccaaaacgttttcatgctcacggtaactaagtgtgatctgtataaaatattacactgattcctcccccgccatgccagatccaggcatttctagactggtagggcataagtaaataatcactctcttcatatcagaccagatggtggttatagtaacactattttgttcgaggtttcactgtgcaggatgccttttaatgcctattggatattatagagcagatgcaatgtgaatgatgactggcagattgtctgcatgaataaaacaaaagagtacacatcctcaatggatgagatagaaaatcgagatctatcactcgtgttgccatttcatcaacagtttaccagataaataagagatttttatttaaaaatgggtgtctgtatcggggccagagtaatgccatatatttttttcttttccttgcaacacacatttttctaccacttactctatgtaagttgtaggtgcttcacattagctgaagacggttatctcagtaaatgcagcagcttcttagcatttggttttgtacctccttttgctctagcctggatgcagctggttcccatggcaatggctgttatgaaaaggtgggacaagaggatatgagacagggcacaagaagaatccagtgcagtccactgtttgtattggtcaattccgggtgcaccctacttcaagtccaagctgccacagagcctttaagatgatgactggccccaagctccttccatccagcaagctattcttgatccctctaaagtcagctctctactaaaaaaaaaaaaaaaagaaataagaaaactcagtggcccagggagtttcaacaaccagtttatctaactgttctacttgttgcagtacaggccacagagacctctacatttattcagtgacctcaaaaataaaaattaaagtttcctccaaataaaaattccttaaatgactttcactaaattttcaggctagctttaatgctggcataaactaaataaacagaatagaattttgtttataaactctccagatttggactattagtcatgagcaacccatacaaataaattttcaaactgaccttttctacccttgccacttcagtgtaagtcatccatgacttctggtcatcccacatactttgtactgacaaacctttaatttgcaaatgaagatgggatgacttaataggtaatttttcatttaagaagtaatatttttgttaagtgccttgtctgactaagttagcaaccaaagttaaatccacagagtataaaaagagttttgtttacacaaaaaaaagaaagaaaggaagaaaaattcttgtccacttcattctttgacaatgcatcagaataatagtgggctataaatagaagatgcaagaatgactaattctgttttgactctatctcttcaatgacaaaggaaacccctctgtacaaacatattaagctaaatcataacagctggactttaggaattttatctagaacatctacatcaaacaactaagggtgccaaccttgaagatgtacaaataactcccagtggaacccagttttataactatcaactcaagggacttgtgatttaaaagaaagatttaaatactgccttgctttaaaagaatactcccttgaaatcatcactgctaataaaatacaggagaaatttaccccaaattactttatcctggaaaaatctgtcttttgtgactgagagagcacacatgcttcatttatagctagaatctttctttctgaaagcttagttatccttcagaaatttgtcagctaaattaagcccttagccatatagagagaagtctgctggcactgcactgggaagagaatgaatgaaagactggattgaattttccatggaagccgacaattaatattgttttctttggtatatccctttctgtccgttgtttttgagctctccaagagaagaaaaaagttaagaagcctgattcagtcatttccaaatctcacttccagtttccatcttatttaagacatgacttaactttaatgtgtgtaacataaacagaatcataaaagggaaagaattagaacagtctggaagagtcggtgtccaaagcaggaaaatgccacagctgatttgccctttttattgttgttggtcttttcgttgtttactgcaaggagaaattatctgttcctctgctgccgcttcctcaccctccattacaatcactgggaattccaatttcacaaagttattacaatacagccacaaataatccatcttgccaagtccatcttcagggccgaagataaagttggagctgagttgctacacacatctggagaaggttcgttacttgtaatcgtgagctgctctgttaatgcacccatgagaaaggggctgacaggctgcatatttctgcaaactgttcccagaaagaaccaatttcctgacttccatgtggtgtcaataatggaggcatgagatggagcagtgcttatgaaatattaaatctgcttacaggaccagctagaagcaaattcagaccacctgtgagaggaagtctagcagtgggtacgcacactttggcacacacatggcacatgtgaatgatatgctctaatctatgcatttgggctcatttgccacaaaacttcctgacagaagtagtgtgtgtgtgtgtgtgtgtgtgtgtgtgtgagagagagagagagagagagagatgcagtaaaacacatttctgcacatttagaactgaaacagttcaaatcactgacattattaaatttactatcataagcagccaaagttcatcttattcatcaggaaaaaagtgactgatgtttcgtggcattagtattagatcattttggttcttgccaataaaaacaaagcattagtgtttcaatgttttaatatcatgatttaattctctcaatgatattaggaccaagaagctcaaccaacgtgaagaccccatcaaaattcttgagtcaaaactatggttctgaaatgagttcaccgtcctgacctcccatttcacagtatatattttatgcttgtgactttccaaatatgggctcttaacattgcaaatgtaaagttttatatgactaacttgtgtttcaagggtttgcctaagtaaatagaaaaacatctgggctctttttactggcaaaagcaagagatatttgacctaagatcagattctgagacttgaacattaacttggtctttccacagaacgtctctaattttccacaactctctgctgagagggttcagcccagtacttttagagaaaggatggacaaagcctgtgtccccctaagacatatgtcccagttggcttctttcaccccaaaactttacccactgttctaatccactcccacctaaacaaaaaggtactactattgcaaggctggaacaaccctccaaagtcagcgtctcagttagactgggggcatctagcccaagatctctccagatgggagggtgtgtaggatactgctttagctgggagtcaggactttcaatctgtcccatcagctcttcaagggcaccatctacaattctagtctgaaattcctttggtttaagataagccccctgcccaggactccctagagtctggaactatagtagtctgcagagtggcattctgggccttgactccctttctgacttggcattgacctctagaagcagaacaggcccaccctccagggacagagtggagattacccagactcaaagactagcagtatggacacctgttcacacacagctctggacggcaccattcccactgcatcccacatgaagggcacacctgcacacacaactccaatgagaggatgcggcctatagctgtgcagcattgcagccactggaatctagtctaacctttcttgaaattttacactaaaatttaaaagcaatcaacctaatccctgatctacttttgtccaagtattttattaaaaatcaactttaacattttttaattgaaagttaaattctatcttggatataaataattatgcttcttcatgacattctgacaaaaatgtagtcacatccaaaggataagaaccaaggctagtttcaatagtcattctcttcacaagttcgataaattcttagaattttagacttttagaacaagattacatattaatatgtctacacgagcacttgtacacgaatgtccatagcagcattattcatagttgccaaaatgtggaaacaattcaagtgtccaccaactggtgaatgcatagacaaagtacagtatgcccatacaatgggctgctattcaacaataagaggaaacacaagtactacagatgactctcaaaaagattatactgtgaaagaagccagacacaaaagacttcatgattccatttttataaaatgcccagaaaaaatgtatagaaacagaaagtagattcctggcagcctgggggttgtggtgggaacaagttgtgactacaaatggacacatcttgttgcagagataaaaatgttccaagtggattatgatgatgatttcccaactctgtaagtttactttaaaaatcactgaactgtagcaaagataaggaatcaacttaagtatccatcaccagatggttggataaagaaaatgtagtgtatattcagccataaaaaaagaacagaatcacatcttttgcagcatcaaagatgaaactggaaatattgtcttaagtgaaataagtcagtgatatggtttggctgtgtccccacccaaatctcaacttgaattgtatctcccagaattcccacgttatgggagagaaccagggggaggtaataatcatgggagctagtctttcccatgctattctcgtgatagtgaataagtctcatgaaaactgatgggtttatcaggggtttctg

SEQ ID NO: 9000 - RNA, 613 nt, Homo sapiens
  source 1..613: mol_type = other RNA
accttcttgtataagcactgtgctaaacgtattcatgcattaacttattcattctcaaacagccgtaagacatagctattaatatcaataccacttaatagatgaggacctcaaactcggtttcagagaggttgaagtcacctgctctcaaggctacccatggaacaagtcccgggttatgatttgtgtccatgctcttcatcactgctgcagaatccctgccaatgtcccaggcatggaggatgtaaagatgagttgtctgtgtccgtcaggtcttccatgaagcagaagacgaaagactgattggaggaaatgcctgtgaaggacaaagggggagggtgctggagaaggtggggagagtcttcagaacacggtacacatctgacaccttttcgctttccatgattcctcttgtatatgtgctctcttgctgcaacaagctaataacctcaacttcggctgcgtgtgtattgctagtaggctttagctgataggctttaagaagacattatctgtgaagcgtgctgtctgtaatagacactcagtaagactccatgccttctcttggctgaccatgctgaatagcagctgtgaaagcccttctgtgagtgga

SEQ ID NO: 9001 - RNA, 4637 nt, Homo sapiens
  source 1..4637: mol_type = other RNA
accttcttgtataagcactgtgctaaactgctttcaaaaattagctggtactaattactctttattctgggttgcaaaatgcccccaaatagtataattcagttttcttgattttaattttttacacattaaaacaattatgtctttggcttgcaagttcaaagtttagtaaaagtcaatgattgtactatatatttccactctgaaatattatagaagtgttcagaaaacataaagtacatatgtggagcttgatgaataaactatagcacatgctagagaaagagcgagaaacagagaaagaataatgttataagacatcaaaatatattttatgtatcaaggtcacaaataatttcaaaattactaaatagtaaaagctgaaaccctccattatcttcttcttagtcattaagaagaaatttattaataatagaataaactaattacaacaggcatttgaaaggataaagagttctggggcaaatatgcttaagacattttaaattttttttgtcagattttaaacttttgttacatcattaaacaagaaaaccccaagttttatgcctgttatttcttgctattagaaatgctcagagcatttatgggtaacccttctgtgacactgaacactttctaccttaacctaaactgcaaagtccttgaaattttgacagctttgtcctcttgattcattttctaccatcgtaccattccttgccaaataccaaacacaagaccatacacatagtggatgtcaatgatgatttactgaatgaaggaagggatgattgaatgaaggaagggatgactgaatgaagaaatgattatgatctcctatgtccctgtgtgttatagcttaaagacattgtgtccataaaaaatgtgtccaaattttgtaggtatatagaagaaaaagaacataaaatgcccataatgttatactaagtccttgattcttattcgacattttaacatttcctcttaaataataacacaggaagttttttgcaatacgataattttctcaactcaagataaaactgtacactattgcctcatactttatatattaataaaaaactgggagcttaaactctccatttttattttatttaatcacctacatcaaaaatacattatttcttcaaatacttaaaatattacacccagggatgataaaacaaatacacaaataatatgatgtatctaaatttgtacatcagttgaatgtgtcatgtatattcagagacacacataaaatttatgtttttatctccttgcctgctaggaattatttccagacctactattttacatcagatctttaccaacagttttccagttgcaaagaccactgtatatatgtatttcccagcagtattagaaacaagaatataattttgcttgacttgtataaccctctgagggctatgaaactgcatttcaagaaatattaactaatgtcatttgaaaggtgatctttaaaatgcatcagaagtgagtgtgggtgtgtttgtgtgtatgtgtatgtgtatgtgtttgtgtgtgtgcgtgtctgtgtgtgtgtgtgatagaaaggtcttgaaaaataactgtattttgggggtgcttctgaagtttgctatatgaacattggccttttttaaaaaataagatgctcagatattttgccaaaatgtgctaaaacaaaatcactcagataatatgagctagtctagagattaataaactctccaatttcaaaagcttatacaaataatgagatgaaaacagacaattttcagccatcaaatatttcaagacttcactctgtttctatgacatattcatcccatacaaaagatttgctaaaggggttgtaatggccttctgggacaggaagaataaggtttctggagaaaatgttaaattaattttgatggtgatgcaaagttaagaaagggttgttaagggatggcttgctgccacagggtggggttttgttttggtatccttttagagcctgcaggtgtttggcactagttaaaatcagggccagctgtgatatttcaatagttctgatattttcctcccaatagatctcagaagtgatgcttcagggtgatgtcttacacctgatatattcgacttgtgtggtacaaatgtgaagactctattaaataacaccaggtttgtgacaccctgtgccctctcttccctaccctcaggtcatggcatccatgacaaagaaaaacactaatcagaggcttcaatcactcatagtttttaattgagcagtttaatcaaagatggtgatatgctggaatcaccaagtaaaaagtcttaagcaaagcctgaaagcagaatggcacattcccttttcattctcaacgtagacaatgatgcttttaatccctctcagtggtgagatatatacctatgtttgcaggaatttgaatagtttctattaaaagctgtattttcttttaagtgtgtttcagttggaaaccctcaaaccacaatgtatttcatgcacatgttcccaagggtatgttaaataggaccatactgaggtcatctagtaagtttttgaaactttttaagaattcctttaatgtactgcacaatcttggcttgattaaaagaagatattttaagaaagcacttggaaaaatgactggctattaaaatctatatgcagataatctatattatacatctataatgcacagagctttccacagataatttgtcattgagaaagacaataaaactcccactctaagggttttgaataaaaactcctcagaactttcagtaaatgcagaccaatccccctccaaccagcctgcagtattcttgattgacttaacagtgtatgcctgcaggatcactttaactgtgcaaaggtctgtcacatataatcagaggataaaaggtagacaatctctcatttatccatgaaaaaaaaatatcatctgttgttttgattgaatcgaaaaatcaagttacctcaatccatgagactatgatgaaattgttaggctagaaatagtttctaccatcaagtaaatttttgttgtctccaagttcaaaccacaaatgaaatgctgtaaatggtctacttgagaagtaggcactcaaatttttctgccgttactgagtctcccaatcctggcttttgttgttgttgttagacataccccttttcactttatcaaagtctccattcctacgccatgttccaggccttgtacttcacccaaagcaatttccagttgaactagcagctgtgctggcacagcgcacatggagagtgggccacacgcgccagtggtgcgttcccacatctgaacagaagtggccgtttccatgcaccaagcgccaagaaactctgcagctcatcagaggcaaaacaagggaggatacctgaggttctgcaaatacattcttcatgttgttgattgggccatacgggactccactgccttcaaaaagatataaccacttgctggtcagttcttcttcaaaccgttcagataatattttaataagctcttttctattgtgtacccgaaggtggttagttttatacttggaattatcaatcaactcaggcaaatccaagatcttgcagacggtggcaaactgctggttatttcctgctccaactacaatatagccatccttggttttaaaagcctggtaaggaacgatactgccatgagctgtaccccaacgttttgcttccttttgaccaataagataatttgcagctatgtgagacaaacacgccacctgggatgacagtaggttacaatcaatgaacagtcctttcccagttttgtatttttgtatcaatccagccataatagctccatatgcatacaggccagtggcaagatcagtcatagctactcctgggcgaactggatctccattctcaggccctgtgatgtgcatcagaccagaaacagccgaggcaacagcatcataaccagctcgctgagaaattggacctgtctgaccataccctgtgatggaacaatagatgatgtgaggagcaatctcgtctatatcttcatatcccaggcccattgcagacagtttgccagggacatagttttccacaaacacatcacaaacagctgcaagctctttgatgattttcaccccttttggatccttgatattaacagcaatactttttttatttcggttaacactgagataatatgtactttctgtcccaacaaaaggtggcccccaagttcgtgtatcatcaccagctcctggtctctccacttttataacttctgctccaagatctcctaaattcatagtagcaaaaggtcccgccaggactcttgttagatccagaatttttaccccttccaatggctttatattgttcatatctgactgcgggcggccagtccacagccccctcccgccgccccggccggagaagaggcaggttctgcgcagagctgccaccctcgccagcgtcgccagcatcgcgtgcgtctcagatggcatcggtcccggtgcaagcggcgaactccgtgcggcgccacccgccgccactggggggcgcccacggacgccgcagaccccgcccccgccgggcggggctgagcactagtcgcctg

SEQ ID NO: 9002 - RNA, 259 nt, Homo sapiens
  source 1..259: mol_type = other RNA
accttcttgtataagcactgtgctaaatgctttcaatgttgattcattgcgtctttacaataccccatcacataggtatgttcagtttcctattagggaaactgaagtgtggagggaagccccttgtccaaggtcactccactagtaagtagcgaagccagtatttgcacctaggcctccaggctccagaaccaacactattagccctaccacagacgacaagtcaggccctcagatatcacactcctggctcatcccc

SEQ ID NO: 9003 - RNA, 4960 nt, Homo sapiens
  source 1..4960: mol_type = other RNA
accttgcatctgcatccccagagggattggcagcagcacctttgatgtaagaatagtcagtgggcttgctgtctttgggtcctcagagaaatggggaggtgaggagatgaactaccccctccacagtctggacagtgcatttctggaggggtggagggagtgaggagcatggacagcccagcgctgggactgcaatgaggactggaggagaagaacgtaggaaacagttgaaggaagcatgaggagctcccagaggggcccggaaacttggtacacaggttgcatcaatcaataaatcaaccaatgcaaagatatctaactctgagacttagaaccattcattcattcattcatttgatcaacaaaattttagtgccatctgtgctgtgccaggcactatatggggcaatgttctggatggagatgattcagaccagtgtcactcccaagccacttaaggcctggtggggaaggatctcagagtatgtgatgaagggcacattttgtgaaggatgggttcttcaagcccatcttgcaagggttgggaaaaccttcatcagggatgttggggggagtattgtggcaggggggaaagccacaagtaaaatgctgagtttggaaagtacacagaggcatttttggggaatagtaagtggatggccaatgtgtgggtgaggaatgagagttaggaccacagagattggctgggccaccttgtggaacacctcccatgtcaagataaggggtttctgtaggtggcttactgtgtgtctggcatgaggtaggcacttcacatgcatctgttaactgtcctgcaaggttgttatccccatcttacaggtggaaggccaggctctgaagggctaggtgacttgccaaatgcagcacaggcaagtcaccgagccaggatttgagcgctaaaagctgagctttggaaaaatgcaaccagaatcaagttgaaggtggggaaatgatcgtgcagcttggtccagcagggaagaaaactaaaaaatgttgattggacttgattcaggaccctgtgggtctaagctcttcaaaccctcaagtctggtccatgaggcggcatcaaatgcgtaggtggccccagctgctgcttttgctagttgtcttccctgggacacttcgatggtgctgtccagcgatcccacgctgttacgccgcccccgcttccctgcatcagagaggtctcgcagggaactgctgagtgcgccccgtttgagcccatcgcctgccccgtaagtgtcctccaggctactgcgggccatcgtcccattcactgagtccttggcccctccaggctgtgaggcgttaggccgcatcatacctttctgcttctccagctccgactccacacggtatttctccatctcctgcacctccgcaatggactcgcgcaggtcggatgtaaagcgcagccggtcctggaggctgggggcattgaagatgatgaggacttttcgctccccaccaggtactgcagacagcaacttgatcccaaactggtaatatgaattctggaagagctgcatgtgcatttccacgagggggaaagactgacggaaactgtacgtcaccaagatcttcttcttctggaaaattttggtgaccacaaggagatcattgaagaggaagacctcccgctgatgcaaccctagcctctgggggcggtttggatctggcacctcgtagagctggcagcagcaaaccagtcgacggtgagggagagacaggactggtttctttccaacaatcatgcgctccacagcctgcacctgggacacatggtcatcgttggtccgcagttcacgcccctggatgcgctggtagatgcccaccaggaggtctcgggggatgtcttcaccattgtcaacccctctcaggttcttgatgaagtcatctagtttcatctttcgttcagctttgacgctgggactgtacatgtcggtattgaggaggatgatggcaaaagcaaggatgaagatggtgtctgggttccggaactggcgcacgagggctgggttacagacacagtaccgctggctgaaggcttcgatgagtcgctccactttctgggcctcaccctgaacccggatatgggactggaacttccggagcgcatcatccagatccatggaggagaagtccatctcatccaccacacagtccaacacgtctctgttgaactgcttctgccggttccctaggaattcccctatcatctgccggctgaggcctttccgctccaggatgaagtgagccactcccaccggtgtgtctgacaggaagccccgctcgatcagatactggatacccttctctggcttcttgttgaagaggttgaggccgattcggtagtgccgcctctggaccacatcattgttgaaagctggcgagtcccagctatgccttgtctcccgctggtaagtctgcttgcacaggccggtagccggaggctcccttagactgtcccgagaagaggagccggagctgcagttgatggtctcattggaattgctggagctctcaaggctctcgttatctccaccatcagagttctcgcctgctgcctcgcacttccccaacctccgacccccagccacaccactgggcccagtgccactgttgggggctggtggcaggggccctggtggggctggggctgggccttcaggggctgggtagtggcggtgtgggatcggggccctgcctggtggccccttgtgcttcagggtcccatgggggctgcagccatcagcctcatacaccagctggcggtggacagagccgcgatctgagcggtcactcaggtccacggagctgtcactaggaggctcaatggtaagcaggggaaggtgggcagcccgcagccggaaatcccggcactccaagcacccgggacccctgcgagtgccttcctcacggctaccgtcttcccgggttcctgatggcactggtggaggaactggcgggagaggggctggcgcccagaactcgggccggccctggggtgggggttctgtgctgggcagtcgctcaggggattgttggggaactgtgtcatccaggtagaggggaagatcactgaaggatgtggctgagctgtcctcttgctgttcctttgactcccgcttctccagctgggctgaccctggctcctcagacatgggccctgacgggtggcagttcagggcttcgtcgatggattcagccagagactttacctgtttggagaaggagtcctcaagttctgtgatgtcattagaaaactctccagatgtggtgacggagcttccaccaccatcgatgcccccaccacaggagcctccatatgggagcccccgttcaagccggtggctccgggcaccagccatggcaccctcgtccagcgaggcaggcttgccctcgaagtacgcggggttctgtgccttctcatactcctcaaaggagaactgcatccgcatgttggaaaggatgatgcggcgggacatgcggctctctgaggctgagctgcgtagccgctcaaagttcttgttcatgcggtactggcggaaggctgtctggatggtcctggcagccctgcggctcaggaaggagcccccatacttcctctccagcatttccaccttcttgtcctgcaggtctgtggagagttcatagctgtccgatagggccttggagcgctttatctcctcctcctcctgcttcctcagggcgacactggctggctggaggcgtgcccgctgagcccagggaaggcccactccagcaggggggccccccatgtggctgctggaggggggcagctggctcagccggtaggggggttggctcccaggactatcaaccgctgtgctcaggtcactgcctggggcatcaccctccacactgctctctgccagcctgcctgagggggtaagcttcatggagtcaaggacctgagtaggacagcaatactggtgtagagtatgagacgctgtggacctgactgttctggaattctcaccatcagattttctctggagggtcgtggccgggctggtgctggtactggtgctgtggcctccgccggcgccgggactggagctcctggatgcgccacggctcagctggccccgctcccgcggtggccgcggccccacgcccaccgccgccgaatagcccgcttccttctcgcggcccgggtgcgccggcccggcctcccgcccgccacgctcgcgacccagggctgggttctcgtggtgcaggtggcactgggccacgtcacgctcgcgggctgtgtaaccggtagtgtcctggagcgggtaggaggcgtcccgctccttgtcccgatacacagcctcccgattctggtaggcgccttcccggttcgggtagcccacgtcccgggccgcctggtggaactggctctcccgcagctcgcggtggtggaactgggtctcgcgcaggttctggtactggctctcgcggcccgggctatcccgcgcgccgtgggggtcccggtgcagctccccgcggtgcagctggctctcctctcgcaggtcgcggttctcctgggtgagctggtccagctggccctccagctcctcgatgcgccgccgctgggtttccagcagctgctgctggctctcgatgatgttgttcagctccagcaggtactccacggcccgatttgggctctcggatcccgggccgcccgggggccccgaccccgcctccatcctggcggcccaggggcaggggaacgggcaggagagccctgtccccgctctctcacggcgccaccctcccccgggcccagccgggggagggggccggcgggacgcgagggcgcgcaccgggcttgagggcccgggggccctagggggcccgggagacagcgctggggccggcggcacggggagcaggagctgaggctgccgccgccaccaccaccaccaca

SEQ ID NO: 9004 - RNA, 1296 nt, Homo sapiens
  source 1..1296: mol_type = other RNA
acgggcagggcagtgcaccctggtgtccagcctggactccacattgcggctccttcctgggaccgcagccgctcagtcctcgttcttctcatgcatgaaggcatccatcttctgggcaaaggtttcagccacaagcagggggaagaccagggaggcgtcagcatagaccttgacgggctgtgcatccacccggatcttgccccaggagacagcctcgtctggtcgggcacctgagtcagagccatcaaactcctgggctgtgttgatgtaaacagcgtagtcggccccgttccgcatgaggttggcattggcaatgtggtgcttgaccacgcccccgcccagaatgatcatcccagtgcacttggcaaagatggcctgtgtgttgatgagcctcaggtcctcaacgatgtccaggaccaggcccgggttcttgtaggaatggaagaagatcatgtcgcccagcgagccgtctgtaagtgcgggactaaacacagggatgtggttcttctgggcccagtaatacacggactctgggttgttgatctccttgcccagccgggcgatcatcttagaaggcgtccactttacaccctctgtgttctgctccatcaccatctggtccagaatgggcatcagccagtcctcaaacttgcagtaattctcattgggcaccagcaggtttccgatcctattgatcccgttctcccggagctccttccccctgaggctaaactcgcccaagtatgtgggcgccaggcacttgatgaggtcttcctccacgccgccagctgtggtcaccaatacgtccaccatgttgtgctgcacaaggtagcgaatggtctcacggatgcctgaactgatgaggttggatgtatatcccaggaaaatggtgcagctggtaagtgggcggcggctctgggtcaggtccgcgtgctggtcttcatcctgtgacagtggttccagcttcttctcgatcatggcattgacttgctgtacagcgcgcccgaagttggttgcttggaagccggtggtgccgaaggcctccagcagtgcgcggtaattcacaccgcggttgaagtcgtagccccggacctgggtgctttcgggcggcaacgtcgagctgtgctttagcacggcggccagcgcccccgctggcgcctcccgttccagggaaccttccatgcgcctatagccggctctcgagtcaaagctgcccctaggccgggcttacggcggcccagaaacgcgttaaaccccgacgcgcgcgtctccgcaagagcacaggaagtagggaac

SEQ ID NO: 9005 - RNA, 2668 nt, Homo sapiens
  source 1..2668: mol_type = other RNA
acgggttaggctcttgggagcttacatctgctccctcctccatattatggctgaagccttagttttacttgtgctcatcaggaatattcatagtctcccacagagggaaagtttctacagctgccctcaggctgttgccagtagcacttgcagaggtgaatgagaaaactttcattggagaccttgggtgctccaagtctgaaaaggcagtagggagaaagctgagcaggaagacagggagggagatcaggaacacacaacgcaccaaaaaatcctacccactgcatagagacaagaaagcttctggtggctcgctactggaaggggggaagcatgtagttttaggatgtaatcaaaagaagtaggagcaaggtaattccattacaaaataaagacctgagcttggaaaagtacaaagggaactattacatctagagattactggctaatctgactacacaagcttgaattcatagtagtggctgacatctaggaaaagtcaggaaattacagacttggaatggtgttgaaaacagatccttggattcagttctcttccccaacgaaaagtattctgcaggcaggagtaaattacctgttctgttggctaaactcataaacatcttttcccccaacctcctgaaaatgagtcagttgcagaatctgaaggccagaagatcttatgtgaaaatacagtcgtttgatctctccatctttccattttggattgcatttctctttttagctggggaagactaacaaagcaaactccaaggtaagggaaaggtaagatgcacaaggaccttaacttacaaaggtcatccggcatagagacgtggtgggtctccatgactccagatggctgggtgtgggtatcaaaacctcaccgccagtcccagtcccctcccccctcaacctgcctcacccctgccccaaagaagcagggatgagtgtgggagggaggacaagcttatattaggtgtaagcgattagggaagaatgacatcacacacgaagaagccaaatatatatatctgtctatgttatagagatgcccacgattatgcttctttttttctctaatggcagcacaggcggcaaagctgggagaaaggctctctgcaggttccaaaatgctggtgcgggatgggctctaggaacagaaagccaagtgccgacggaaactgagagcaccccagctctaccaatggcagtcctctagaaaaggcagtaagaacggaagcggtgaggggtgcagctgaagaccgccagggctgcaccccacttaatggctttcccctcatgccttgggggggtctccactgggtggaggaaggaagccagggtgggatggaaagccccctcttctgtggcaaccctgaagtcagcctcttggaactgagggttgacctcagcagagagtctcctgttgacccttgggttgaaagaatggggagtggaggtgactgtgtgttcatgcctctctcttgctctctcaccattatacctggatggctgctggaattccgagatgaagatgaagtttttctctagagttatgactgatggttgaagcaataatttggaaatcctggcgatttattgcattagaaaacaaaaccattaaagcactgaagacagccctttagtgtccctgccaaggagatgaagctgaagtgcaaccccagttgcactcaaccttgggttctttactgaacggttccatcgtccgcatccatccatagtccataggtccgtgtctgctgtgtggaggaagagtctgcccgcacggcatgcacatgcgcggtgagctgcaacacagtgtggctggcgggaggctgctactccatgccgctccggagtatctggttggctgcaatcagcatgacactgatgatgaaggccatagcaaaggcgcatatgaggctcttccggacgcaggtctgtctgttctgcttctgggaatgcactccttcaaactctgtttggcagttccccgaggtctcattcaggctctcttcctcattgataatgatgttctcaatgtccttcatcgttaggtggtctcggaaggcatgatagagaatgtgcttcaactcttccagagttatcctttgcatgtcaaactgccagaatatgctgtctatcgtgttcccaagaaaaccatcgcgaccttctgaagacaccagtttggggccaagaatggtcatgaattcatcaaaatccacctggccatccccgtccatgtccaagcgctgcatgatgatggccagctccacctcgcttggcatgtaccccaaagagcgcatggccatgcccagctcctgcttggagatgaagccgttcccatcccggtccagaacccgaaaggcctctcggatttcatcgagctcctccacggagatattagccagctgttcgctgtcactgccagcagagagcgatcggttgaggtaattccccttgtacaacaagccggcggtcacatggtggaacggcatcttttccatcacagtgaccacagtggaggctcaggctgagaatcccaccgcataaaggttaagatgacaaaggcaaacggattgctgtgcccggcttcataggcaataaatcccatgtgtctttcatccttcccaccctctccccggtgagtctatttccatgatga

SEQ ID NO: 9006 - RNA, 3156 nt, Homo sapiens
  source 1..3156: mol_type = other RNA
acgggttaggctcttgggagcttacatctgctccctcctccatattatggctgaagccttagttttacttgtgctcatcaggaatattcatagtctcccacagagggaaagtttctacagctgccctcaggctgttgccagtagcacttgcagaggtgaatgagaaaactttcattggagaccttgggtgctccaagtctgaaaaggcagtagggagaaagctgagcaggaagacagggagggagatcaggaacacacaacgcaccaaaaaatcctacccactgcatagagacaagaaagcttctggtggctcgctactggaaggggggaagcatgtagttttaggatgtaatcaaaagaagtaggagcaaggtaattccattacaaaataaagacctgagcttggaaaagtacaaagggaactattacatctagagattactggctaatctgactacacaagcttgaattcatagtagtggctgacatctaggaaaagtcaggaaattacagacttggaatggtgttgaaaacagatccttggattcagttctcttccccaacgaaaagtattctgcaggcaggagtaaattacctgttctgttggctaaactcataaacatcttttcccccaacctcctgaaaatgagtcagttgcagaatctgaaggccagaagatcttatgtgaaaatacagtcgtttgatctctccatctttccattttggattgcatttctctttttagctggggaagactaacaaagcaaactccaaggtaagggaaaggtaagatgcacaaggaccttaacttacaaaggtcatccggcatagagacgtggtgggtctccatgactccagatggctgggtgtgggtatcaaaacctcaccgccagtcccagtcccctcccccctcaacctgcctcacccctgccccaaagaagcagggatgagtgtgggagggaggacaagcttatattaggtgtaagcgattagggaagaatgacatcacacacgaagaagccaaatatatatatctgtctatgttatagagatgcccacgattatgcttctttttttctctaatggcagcacaggcggcaaagctgggagaaaggctctctgcaggttccaaaatgctggtgcgggatgggctctaggaacagaaagccaagtgccgacggaaactgagagcaccccagctctaccaatggcagtcctctagaaaaggcagtaagaacggaagcggtgaggggtgcagctgaagaccgccagggctgcaccccacttaatggctttcccctcatgccttgggggggtctccactgggtggaggaaggaagccagggtgggatggaaagccccctcttctgtggcaaccctgaagtcagcctcttggaactgagggttgacctcagcagagagtctcctgttgacccttgggttgaaagaatggggagtggaggtgactgtgtgttcatgcctctctcttgctctctcaccattatacctggatggctgctggaattccgagatgaagatgaagtttttctctagagttatgactgatggttgaagcaataatttggaaatcctggcgatttattgcattagaaaacaaaaccattaaagcactgaagacagccctttagtgtccctgccaaggagatgaagctgaagtgcaaccccagttgcactcaaccttgggttctttactgaacggttccatcgtccgcatccatccatagtccataggtccgtgtctgctgtgtggaggaagagtctgcccgcacggcatgcacatgcgcggtgagctgcaacacagtgtggctggcgggaggctgctactccatgccgctccggagtatctggttggctgcaatcagcatgacactgatgatgaaggccatagcaaaggcgcatatgaggctcttccggacgcaggtctgtctgttctgcttctgggaatgcactccttcaaactctgtttggcagttccccgaggtctcattcaggctctcttcctcattgataatgatgttctcaatgtccttcatcgttaggtggtctcggaaggcatgatagagaatgtgcttcaactcttccagagttatcctttgcatgtcaaactgccagaatatgctgtctatcgtgttcccaagaaaaccatcgcgaccttctgaagacaccagtttggggccaagaatggtcatgaattcatcaaaatccacctggccatccccgtccatgtccaagcgctgcatgatgatggccagctccacctcgcttggcatgtaccccaaagagcgcatggccatgcccagctcctgcttggagatgaagccgttcccatcccggtccagaacccgaaaggcctctcggatttcatcgagctcctccacggagatattagccagctgttcgctgtcactgccagcagagagcgatcggttgaggtaattccccttgtacaacaagccggcggtcacatggtggaacggcatcttttcccaggtggggaagtcgggggcctggctcctcggcggctcctctccccctccgagggctcctccgtccccctttttctcattctcgggcttcccctctccgggttgctctggcagccgcatcgggggtccagggcgatgttctcagagagagttagaagctcatcaaaggaacgtcagcgaaggcactgagactctcctgctgatctcgggggaaattctccaagatccatggctgggagttaaggagaatctctaagccatcaggaaggagcagggcactgcagctcctcagaatgatggaccggggcgagctttaattaacagggtctgatgcctcttcttttttggtaactgagcagatttaaagggctagagtcccaatttgaagggtgccagtgctgctgccgtggctgctgccgtgtctgctctggctgctgctcctgctgctgggaaagcttcctgcagccctctcactccagcaagaaaacggggctgagaaggtggaaaagtgcccccagaaacaccggagtctctcgggctgcatggtttgaatcggaaccacagggctgtggacccacgcactgcctaccctaggaagtaccaaggtcctgctcgctgtcttccagaccgagggaaagagcggggctcc

SEQ ID NO: 9007 - RNA, 3373 nt, Homo sapiens
  source 1..3373: mol_type = other RNA
acgggttaggctcttgggagcttacatctgctccctcctccatattatggctgaagccttagttttacttgtgctcatcaggaatattcatagtctcccacagagggaaagtttctacagctgccctcaggctgttgccagtagcacttgcagaggtgaatgagaaaactttcattggagaccttgggtgctccaagtctgaaaaggcagtagggagaaagctgagcaggaagacagggagggagatcaggaacacacaacgcaccaaaaaatcctacccactgcatagagacaagaaagcttctggtggctcgctactggaaggggggaagcatgtagttttaggatgtaatcaaaagaagtaggagcaaggtaattccattacaaaataaagacctgagcttggaaaagtacaaagggaactattacatctagagattactggctaatctgactacacaagcttgaattcatagtagtggctgacatctaggaaaagtcaggaaattacagacttggaatggtgttgaaaacagatccttggattcagttctcttccccaacgaaaagtattctgcaggcaggagtaaattacctgttctgttggctaaactcataaacatcttttcccccaacctcctgaaaatgagtcagttgcagaatctgaaggccagaagatcttatgtgaaaatacagtcgtttgatctctccatctttccattttggattgcatttctctttttagctggggaagactaacaaagcaaactccaaggtaagggaaaggtaagatgcacaaggaccttaacttacaaaggtcatccggcatagagacgtggtgggtctccatgactccagatggctgggtgtgggtatcaaaacctcaccgccagtcccagtcccctcccccctcaacctgcctcacccctgccccaaagaagcagggatgagtgtgggagggaggacaagcttatattaggtgtaagcgattagggaagaatgacatcacacacgaagaagccaaatatatatatctgtctatgttatagagatgcccacgattatgcttctttttttctctaatggcagcacaggcggcaaagctgggagaaaggctctctgcaggttccaaaatgctggtgcgggatgggctctaggaacagaaagccaagtgccgacggaaactgagagcaccccagctctaccaatggcagtcctctagaaaaggcagtaagaacggaagcggtgaggggtgcagctgaagaccgccagggctgcaccccacttaatggctttcccctcatgccttgggggggtctccactgggtggaggaaggaagccagggtgggatggaaagccccctcttctgtggcaaccctgaagtcagcctcttggaactgagggttgacctcagcagagagtctcctgttgacccttgggttgaaagaatggggagtggaggtgactgtgtgttcatgcctctctcttgctctctcaccattatacctggatggctgctggaattccgagatgaagatgaagtttttctctagagttatgactgatggttgaagcaataatttggaaatcctggcgatttattgcattagaaaacaaaaccattaaagcactgaagacagccctttagtgtccctgccaaggagatgaagctgaagtgcaaccccagttgcactcaaccttgggttctttactgaacggttccatcgtccgcatccatccatagtccataggtccgtgtctgctgtgtggaggaagagtctgcccgcacggcatgcacatgcgcggtgagctgcaacacagtgtggctggcgggaggctgctactccatgccgctccggagtatctggttggctgcaatcagcatgacactgatgatgaaggccatagcaaaggcgcatatgaggctcttccggacgcaggtctgtctgttctgcttctgggaatgcactccttcaaactctgtttggcagttccccgaggtctcattcaggctctcttcctcattgataatgatgttctcaatgtccttcatcgttaggtggtctcggaaggcatgatagagaatgtgcttcaactcttccagagttatcctttgcatgtcaaactgccagaatatgctgtctatcgtgttcccaagaaaaccatcgcgaccttctgaagacaccagtttggggccaagaatggtcatgaattcatcaaaatccacctggccatccccgtccatgtccaagcgctgcatgatgatggccagctccacctcgcttggcatgtaccccaaagagcgcatggccatgcccagctcctgcttggagatgaagccgttcccatcccggtccagaacccgaaaggcctctcggatttcatcgagctcctccacggagatattagccagctgttcgctgtcactgccagcagagagcgatcggttgaggtaattccccttgtacaacaagccggcggtcacatggtggaacggcatcttttcccaggtggggaagtcgggggcctggctcctcggcggctcctctccccctccgagggctcctccgtccccctttttctcattctcgggcttcccctctccgggttgctctggcagccgcatcgggggtccagggcgatgttctcagagagagttagaagctcatcaaaggaacgtcagcgaaggcactgagactctgtgtgcggaatttattccttctgctgggttgttggtctcgccgactttaagaataaaaccacggacctcgcggtgagtgttacagctcttaaagatggcgcgtccggagtcgtctgctcctcccggtgggcttgcggtcttgctgacttcaagaacgaagacgcagaccgcggccgtgagctttaaaggtggcgcggacccagagtaagcagtaagctcctgctgatctcgggggaaattctccaagatccatggctgggagttaaggagaatctctaagccatcaggaaggagcagggcactgcagctcctcagaatgatggaccggggcgagctttaattaacagggtctgatgcctcttcttttttggtaactgagcagatttaaagggctagagtcccaatttgaagggtgccagtgctgctgccgtggctgctgccgtgtctgctctggctgctgctcctgctgctgggaaagcttcctgcagccctctcactccagcaagaaaacggggctgagaaggtggaaaagtgcccccagaaacaccggagtctctcgggctgcatggtttgaatcggaaccacagggctgtggacccacgcactgcctaccctaggaagtaccaaggtcctgctcgctgtcttccagaccgagggaaagagcggggctc

SEQ ID NO: 9008 - RNA, 2981 nt, Homo sapiens
  source 1..2981: mol_type = other RNA
acgggttaggctcttgggagcttacatctgctccctcctccatattatggctgaagccttagttttacttgtgctcatcaggaatattcatagtctcccacagagggaaagtttctacagctgccctcaggctgttgccagtagcacttgcagaggtgaatgagaaaactttcattggagaccttgggtgctccaagtctgaaaaggcagtagggagaaagctgagcaggaagacagggagggagatcaggaacacacaacgcaccaaaaaatcctacccactgcatagagacaagaaagcttctggtggctcgctactggaaggggggaagcatgtagttttaggatgtaatcaaaagaagtaggagcaaggtaattccattacaaaataaagacctgagcttggaaaagtacaaagggaactattacatctagagattactggctaatctgactacacaagcttgaattcatagtagtggctgacatctaggaaaagtcaggaaattacagacttggaatggtgttgaaaacagatccttggattcagttctcttccccaacgaaaagtattctgcaggcaggagtaaattacctgttctgttggctaaactcataaacatcttttcccccaacctcctgaaaatgagtcagttgcagaatctgaaggccagaagatcttatgtgaaaatacagtcgtttgatctctccatctttccattttggattgcatttctctttttagctggggaagactaacaaagcaaactccaaggtaagggaaaggtaagatgcacaaggaccttaacttacaaaggtcatccggcatagagacgtggtgggtctccatgactccagatggctgggtgtgggtatcaaaacctcaccgccagtcccagtcccctcccccctcaacctgcctcacccctgccccaaagaagcagggatgagtgtgggagggaggacaagcttatattaggtgtaagcgattagggaagaatgacatcacacacgaagaagccaaatatatatatctgtctatgttatagagatgcccacgattatgcttctttttttctctaatggcagcacaggcggcaaagctgggagaaaggctctctgcaggttccaaaatgctggtgcgggatgggctctaggaacagaaagccaagtgccgacggaaactgagagcaccccagctctaccaatggcagtcctctagaaaaggcagtaagaacggaagcggtgaggggtgcagctgaagaccgccagggctgcaccccacttaatggctttcccctcatgccttgggggggtctccactgggtggaggaaggaagccagggtgggatggaaagccccctcttctgtggcaaccctgaagtcagcctcttggaactgagggttgacctcagcagagagtctcctgttgacccttgggttgaaagaatggggagtggaggtgactgtgtgttcatgcctctctcttgctctctcaccattatacctggatggctgctggaattccgagatgaagatgaagtttttctctagagttatgactgatggttgaagcaataatttggaaatcctggcgatttattgcattagaaaacaaaaccattaaagcactgaagacagccctttagtgtccctgccaaggagatgaagctgaagtgcaaccccagttgcactcaaccttgggttctttactgaacggttccatcgtccgcatccatccatagtccataggtccgtgtctgctgtgtggaggaagagtctgcccgcacggcatgcacatgcgcggtgagctgcaacacagtgtggctggcgggaggctgctactccatgccgctccggagtatctggttggctgcaatcagcatgacactgatgatgaaggccatagcaaaggcgcatatgaggctcttccggacgcaggtctgtctgttctgcttctgggaatgcactccttcaaactctgtttggcagttccccgaggtctcattcaggctctcttcctcattgataatgatgttctcaatgtccttcatcgttaggtggtctcggaaggcatgatagagaatgtgcttcaactcttccagagttatcctttgcatgtcaaactgccagaatatgctgtctatcgtgttcccaagaaaaccatcgcgaccttctgaagacaccagtttggggccaagaatggtcatgaattcatcaaaatccacctggccatccccgtccatgtccaagcgctgcatgatgatggccagctccacctcgcttggcatgtaccccaaagagcgcatggccatgcccagctcctgcttggagatgaagccgttcccatcccggtccagaacccgaaaggcctctcggatttcatcgagctcctccacggagatattagccagctgttcgctgtcactgccagcagagagcgatcggttgaggtaattccccttgtacaacaagccggcggtcacatggtggaacggcatcttttcccaggtggggaagtcgggggcctggctcctcggcggctcctctccccctccgagggctcctccgtccccctttttctcattctcgggcttcccctctccgggttgctctggcagccgcatcgggggtccagggcgatgttctcagagagagttagaagctcatcaaaggaacgtcagcgaaggcactgagactctgtgtgcggaatttattccttctgctgggttgttggtctcgccgactttaagaataaaaccacggacctcgcggtgagtgttacagctcttaaagatggcgcgtccggagtcgtctgctcctcccggtgggcttgcggtcttgctgacttcaagaacgaagacgcagaccgcggccgtgagctttaaaggtggcgcggacccagagtaagcagtaagctttattaagaagcaggaaagaaaaaaacacaaactcaagcggatagcaccccagcgagcttc

SEQ ID NO: 9009 - RNA, 2979 nt, Homo sapiens
  source 1..2979: mol_type = other RNA
acgggttaggctcttgggagcttacatctgctccctcctccatattatggctgaagccttagttttacttgtgctcatcaggaatattcatagtctcccacagagggaaagtttctacagctgccctcaggctgttgccagtagcacttgcagaggtgaatgagaaaactttcattggagaccttgggtgctccaagtctgaaaaggcagtagggagaaagctgagcaggaagacagggagggagatcaggaacacacaacgcaccaaaaaatcctacccactgcatagagacaagaaagcttctggtggctcgctactggaaggggggaagcatgtagttttaggatgtaatcaaaagaagtaggagcaaggtaattccattacaaaataaagacctgagcttggaaaagtacaaagggaactattacatctagagattactggctaatctgactacacaagcttgaattcatagtagtggctgacatctaggaaaagtcaggaaattacagacttggaatggtgttgaaaacagatccttggattcagttctcttccccaacgaaaagtattctgcaggcaggagtaaattacctgttctgttggctaaactcataaacatcttttcccccaacctcctgaaaatgagtcagttgcagaatctgaaggccagaagatcttatgtgaaaatacagtcgtttgatctctccatctttccattttggattgcatttctctttttagctggggaagactaacaaagcaaactccaaggtaagggaaaggtaagatgcacaaggaccttaacttacaaaggtcatccggcatagagacgtggtgggtctccatgactccagatggctgggtgtgggtatcaaaacctcaccgccagtcccagtcccctcccccctcaacctgcctcacccctgccccaaagaagcagggatgagtgtgggagggaggacaagcttatattaggtgtaagcgattagggaagaatgacatcacacacgaagaagccaaatatatatatctgtctatgttatagagatgcccacgattatgcttctttttttctctaatggcagcacaggcggcaaagctgggagaaaggctctctgcaggttccaaaatgctggtgcgggatgggctctaggaacagaaagccaagtgccgacggaaactgagagcaccccagctctaccaatggcagtcctctagaaaaggcagtaagaacggaagcggtgaggggtgcagctgaagaccgccagggctgcaccccacttaatggctttcccctcatgccttgggggggtctccactgggtggaggaaggaagccagggtgggatggaaagccccctcttctgtggcaaccctgaagtcagcctcttggaactgagggttgacctcagcagagagtctcctgttgacccttgggttgaaagaatggggagtggaggtgactgtgtgttcatgcctctctcttgctctctcaccattatacctggatggctgctggaattccgagatgaagatgaagtttttctctagagttatgactgatggttgaagcaataatttggaaatcctggcgatttattgcattagaaaacaaaaccattaaagcactgaagacagccctttagtgtccctgccaaggagatgaagctgaagtgcaaccccagttgcactcaaccttgggttctttactgaacggttccatcgtccgcatccatccatagtccataggtccgtgtctgctgtgtggaggaagagtctgcccgcacggcatgcacatgcgcggtgagctgcaacacagtgtggctggcgggaggctgctactccatgccgctccggagtatctggttggctgcaatcagcatgacactgatgatgaaggccatagcaaaggcgcatatgaggctcttccggacgcaggtctgtctgttctgcttctgggaatgcactccttcaaactctgtttggcagttccccgaggtctcattcaggctctcttcctcattgataatgatgttctcaatgtccttcatcgttaggtggtctcggaaggcatgatagagaatgtgcttcaactcttccagagttatcctttgcatgtcaaactgccagaatatgctgtctatcgtgttcccaagaaaaccatcgcgaccttctgaagacaccagtttggggccaagaatggtcatgaattcatcaaaatccacctggccatccccgtccatgtccaagcgctgcatgatgatggccagctccacctcgcttggcatgtaccccaaagagcgcatggccatgcccagctcctgcttggagatgaagccgttcccatcccggtccagaacccgaaaggcctctcggatttcatcgagctcctccacggagatattagccagctgttcgctgtcactgccagcagagagcgatcggttgaggtaattccccttgtacaacaagccggcggtcacatggtggaacggcatcttttcccatcatgtagaatcagtgggagccctgagcttatttttctgcaactggatggtcccatccgggggtgctcctgctgatctcgggggaaattctccaagatccatggctgggagttaaggagaatctctaagccatcaggaaggagcagggcactgcagctcctcagaatgatggaccggggcgagctttaattaacagggtctgatgcctcttcttttttggtaactgagcagatttaaagggctagagtcccaatttgaagggtgccagtgctgctgccgtggctgctgccgtgtctgctctggctgctgctcctgctgctgggaaagcttcctgcagccctctcactccagcaagaaaacggggctgagaaggtggaaaagtgcccccagaaacaccggagtctctcgggctgcatggtttgaatcggaaccacagggctgtggacccacgcactgcctaccctaggaa

SEQ ID NO: 9010 - RNA, 3513 nt, Homo sapiens
  source 1..3513: mol_type = other RNA
acgggttaggctcttgggagcttacatctgctccctcctccatattatggctgaagccttagttttacttgtgctcatcaggaatattcatagtctcccacagagggaaagtttctacagctgccctcaggctgttgccagtagcacttgcagaggtgaatgagaaaactttcattggagaccttgggtgctccaagtctgaaaaggcagtagggagaaagctgagcaggaagacagggagggagatcaggaacacacaacgcaccaaaaaatcctacccactgcatagagacaagaaagcttctggtggctcgctactggaaggggggaagcatgtagttttaggatgtaatcaaaagaagtaggagcaaggtaattccattacaaaataaagacctgagcttggaaaagtacaaagggaactattacatctagagattactggctaatctgactacacaagcttgaattcatagtagtggctgacatctaggaaaagtcaggaaattacagacttggaatggtgttgaaaacagatccttggattcagttctcttccccaacgaaaagtattctgcaggcaggagtaaattacctgttctgttggctaaactcataaacatcttttcccccaacctcctgaaaatgagtcagttgcagaatctgaaggccagaagatcttatgtgaaaatacagtcgtttgatctctccatctttccattttggattgcatttctctttttagctggggaagactaacaaagcaaactccaaggtaagggaaaggtaagatgcacaaggaccttaacttacaaaggtcatccggcatagagacgtggtgggtctccatgactccagatggctgggtgtgggtatcaaaacctcaccgccagtcccagtcccctcccccctcaacctgcctcacccctgccccaaagaagcagggatgagtgtgggagggaggacaagcttatattaggtgtaagcgattagggaagaatgacatcacacacgaagaagccaaatatatatatctgtctatgttatagagatgcccacgattatgcttctttttttctctaatggcagcacaggcggcaaagctgggagaaaggctctctgcaggttccaaaatgctggtgcgggatgggctctaggaacagaaagccaagtgccgacggaaactgagagcaccccagctctaccaatggcagtcctctagaaaaggcagtaagaacggaagcggtgaggggtgcagctgaagaccgccagggctgcaccccacttaatggctttcccctcatgccttgggggggtctccactgggtggaggaaggaagccagggtgggatggaaagccccctcttctgtggcaaccctgaagtcagcctcttggaactgagggttgacctcagcagagagtctcctgttgacccttgggttgaaagaatggggagtggaggtgactgtgtgttcatgcctctctcttgctctctcaccattatacctggatggctgctggaattccgagatgaagatgaagtttttctctagagttatgactgatggttgaagcaataatttggaaatcctggcgatttattgcattagaaaacaaaaccattaaagcactgaagacagccctttagtgtccctgccaaggagatgaagctgaagtgcaaccccagttgcactcaaccttgggttctttactgaacggttccatcgtccgcatccatccatagtccataggtccgtgtctgctgtgtggaggaagagtctgcccgcacggcatgcacatgcgcggtgagctgcaacacagtgtggctggcgggaggctgctactccatgccgctccggagtatctggttggctgcaatcagcatgacactgatgatgaaggccatagcaaaggcgcatatgaggctcttccggacgcaggtctgtctgttctgcttctgggaatgcactccttcaaactctgtttggcagttccccgaggtctcattcaggctctcttcctcattgataatgatgttctcaatgtccttcatcgttaggtggtctcggaaggcatgatagagaatgtgcttcaactcttccagagttatcctttgcatgtcaaactgccagaatatgctgtctatcgtgttcccaagaaaaccatcgcgaccttctgaagacaccagtttggggccaagaatggtcatgaattcatcaaaatccacctggccatccccgtccatgtccaagcgctgcatgatgatggccagctccacctcgcttggcatgtaccccaaagagcgcatggccatgcccagctcctgcttggagatgaagccgttcccatcccggtccagaacccgaaaggcctctcggatttcatcgagctcctccacggagatattagccagctgttcgctgtcactgccagcagagagcgatcggttgaggtaattccccttgtacaacaagccggcggtcacatggtggaacggcatcttttcccatcatgtagaatcagtgggagccctgagcttatttttctgcaactggatggtcccatccgggggtgctctgggtttccaagtactaagccgtgaccctgtgcaacatctctgtgacctggctacatctctgtttcttcatctgtaaaatgggagaaataaagcagatgacacctactaagcactaagctagtttgcctgctgagatggaatatgtgtttatgtgtatgcatataaaatgaatcatcagccacagatcagattaaaaagcagagcaactggttttccgaaccagcagtaggaatgctggaggctgagacgccacatcagtgttcagtacagatgtttgaggttttcttaccaggctataaaaatgtttacacagtaattaggcctgttatcagtacacaaacagattacaatttgcagaatgaatgaacagctcaaaaaccctctcggttttcatgaggttcggagcattttcctaattcttgggtttacaaaaataaattcggtttccaataacaaggagccacagctgagtgtaggggaaagggctctggggtgtgaaatgaactctgtttgacagtgcacatgtcactcagtctctctgactgagtctccccatctgtcaaatgagctaaccaaggttcctcttctcctttaaattccatggttctattactttgcagtcaatgtcttctaaacacatattcattcttttcaccacaaaaggatatgtttagttaatgatttttaaggtagtaattctgctgaatcacatgagactccaatccaacactattcagtcatattgagactgagtttgtggcagttaattcctgacaatgaagcccccaagcccagtctgtaggatgagaccacaaggtcaacttgggctttatgtgaacatccagctcttccagaacacatcaatggttctgagtaacacttgattgaggctgggtgcagtggctcacgcctgtaatcccagcactttgggagg

SEQ ID NO: 9011 - RNA, 2645 nt, Homo sapiens
  source 1..2645: mol_type = other RNA
acgggttaggctcttgggagcttacatctgctccctcctccatattatggctgaagccttagttttacttgtgctcatcaggaatattcatagtctcccacagagggaaagtttctacagctgccctcaggctgttgccagtagcacttgcagaggtgaatgagaaaactttcattggagaccttgggtgctccaagtctgaaaaggcagtagggagaaagctgagcaggaagacagggagggagatcaggaacacacaacgcaccaaaaaatcctacccactgcatagagacaagaaagcttctggtggctcgctactggaaggggggaagcatgtagttttaggatgtaatcaaaagaagtaggagcaaggtaattccattacaaaataaagacctgagcttggaaaagtacaaagggaactattacatctagagattactggctaatctgactacacaagcttgaattcatagtagtggctgacatctaggaaaagtcaggaaattacagacttggaatggtgttgaaaacagatccttggattcagttctcttccccaacgaaaagtattctgcaggcaggagtaaattacctgttctgttggctaaactcataaacatcttttcccccaacctcctgaaaatgagtcagttgcagaatctgaaggccagaagatcttatgtgaaaatacagtcgtttgatctctccatctttccattttggattgcatttctctttttagctggggaagactaacaaagcaaactccaaggtaagggaaaggtaagatgcacaaggaccttaacttacaaaggtcatccggcatagagacgtggtgggtctccatgactccagatggctgggtgtgggtatcaaaacctcaccgccagtcccagtcccctcccccctcaacctgcctcacccctgccccaaagaagcagggatgagtgtgggagggaggacaagcttatattaggtgtaagcgattagggaagaatgacatcacacacgaagaagccaaatatatatatctgtctatgttatagagatgcccacgattatgcttctttttttctctaatggcagcacaggcggcaaagctgggagaaaggctctctgcaggttccaaaatgctggtgcgggatgggctctaggaacagaaagccaagtgccgacggaaactgagagcaccccagctctaccaatggcagtcctctagaaaaggcagtaagaacggaagcggtgaggggtgcagctgaagaccgccagggctgcaccccacttaatggctttcccctcatgccttgggggggtctccactgggtggaggaaggaagccagggtgggatggaaagccccctcttctgtggcaaccctgaagtcagcctcttggaactgagggttgacctcagcagagagtctcctgttgacccttgggttgaaagaatggggagtggaggtgactgtgtgttcatgcctctctcttgctctctcaccattatacctggatggctgctggaattccgagatgaagatgaagtttttctctagagttatgactgatggttgaagcaataatttggaaatcctggcgatttattgcattagaaaacaaaaccattaaagcactgaagacagccctttagtgtccctgccaaggagatgaagctgaagtgcaaccccagttgcactcaaccttgggttctttactgaacggttccatcgtccgcatccatccatagtccataggtccgtgtctgctgtgtggaggaagagtctgcccgcacggcatgcacatgcgcggtgagctgcaacacagtgtggctggcgggaggctgctactccatgccgctccggagtatctggttggctgcaatcagcatgacactgatgatgaaggccatagcaaaggcgcatatgaggctcttccggacgcaggtctgtctgttctgcttctgggaatgcactccttcaaactctgtttggcagttccccgaggtctcattcaggctctcttcctcattgataatgatgttctcaatgtccttcatcgttaggtggtctcggaaggcatgatagagaatgtgcttcaactcttccagagttatcctttgcatgtcaaactgccagaatatgctgtctatcgtgttcccaagaaaaccatcgcgaccttctgaagacaccagtttggggccaagaatggtcatgaattcatcaaaatccacctggccatccccgtccatgtccaagcgctgcatgatgatggccagctccacctcgcttggcatgtaccccaaagagcgcatggccatgcccagctcctgcttggagatgaagccgttcccatcccggtccagaacccgaaaggcctctcggatttcatcgagctcctccacggagatattagccagctgttcgctgtcactgccagcagagagcgatcggttgaggtaattccccttgtacaacaagccggcggtcacatggtggaacggcatcttttcccctagcgcccgccgccttcactacttcatcccaggtgcccacaccctagatccacgattacacctgagcccagggggaaggcggggcgccgaagtggaggggccaatggccgaaactgcggggaccagcattccgcg

SEQ ID NO: 9012 - RNA, 2610 nt, Homo sapiens
  source 1..2610: mol_type = other RNA
acgggttaggctcttgggagcttacatctgctccctcctccatattatggctgaagccttagttttacttgtgctcatcaggaatattcatagtctcccacagagggaaagtttctacagctgccctcaggctgttgccagtagcacttgcagaggtgaatgagaaaactttcattggagaccttgggtgctccaagtctgaaaaggcagtagggagaaagctgagcaggaagacagggagggagatcaggaacacacaacgcaccaaaaaatcctacccactgcatagagacaagaaagcttctggtggctcgctactggaaggggggaagcatgtagttttaggatgtaatcaaaagaagtaggagcaaggtaattccattacaaaataaagacctgagcttggaaaagtacaaagggaactattacatctagagattactggctaatctgactacacaagcttgaattcatagtagtggctgacatctaggaaaagtcaggaaattacagacttggaatggtgttgaaaacagatccttggattcagttctcttccccaacgaaaagtattctgcaggcaggagtaaattacctgttctgttggctaaactcataaacatcttttcccccaacctcctgaaaatgagtcagttgcagaatctgaaggccagaagatcttatgtgaaaatacagtcgtttgatctctccatctttccattttggattgcatttctctttttagctggggaagactaacaaagcaaactccaaggtaagggaaaggtaagatgcacaaggaccttaacttacaaaggtcatccggcatagagacgtggtgggtctccatgactccagatggctgggtgtgggtatcaaaacctcaccgccagtcccagtcccctcccccctcaacctgcctcacccctgccccaaagaagcagggatgagtgtgggagggaggacaagcttatattaggtgtaagcgattagggaagaatgacatcacacacgaagaagccaaatatatatatctgtctatgttatagagatgcccacgattatgcttctttttttctctaatggcagcacaggcggcaaagctgggagaaaggctctctgcaggttccaaaatgctggtgcgggatgggctctaggaacagaaagccaagtgccgacggaaactgagagcaccccagctctaccaatggcagtcctctagaaaaggcagtaagaacggaagcggtgaggggtgcagctgaagaccgccagggctgcaccccacttaatggctttcccctcatgccttgggggggtctccactgggtggaggaaggaagccagggtgggatggaaagccccctcttctgtggcaaccctgaagtcagcctcttggaactgagggttgacctcagcagagagtctcctgttgacccttgggttgaaagaatggggagtggaggtgactgtgtgttcatgcctctctcttgctctctcaccattatacctggatggctgctggaattccgagatgaagatgaagtttttctctagagttatgactgatggttgaagcaataatttggaaatcctggcgatttattgcattagaaaacaaaaccattaaagcactgaagacagccctttagtgtccctgccaaggagatgaagctgaagtgcaaccccagttgcactcaaccttgggttctttactgaacggttccatcgtccgcatccatccatagtccataggtccgtgtctgctgtgtggaggaagagtctgcccgcacggcatgcacatgcgcggtgagctgcaacacagtgtggctggcgggaggctgctactccatgccgctccggagtatctggttggctgcaatcagcatgacactgatgatgaaggccatagcaaaggcgcatatgaggctcttccggacgcaggtctgtctgttctgcttctgggaatgcactccttcaaactctgtttggcagttccccgaggtctcattcaggctctcttcctcattgataatgatgttctcaatgtccttcatcgttaggtggtctcggaaggcatgatagagaatgtgcttcaactcttccagagttatcctttgcatgtcaaactgccagaatatgctgtctatcgtgttcccaagaaaaccatcgcgaccttctgaagacaccagtttggggccaagaatggtcatgaattcatcaaaatccacctggccatccccgtccatgtccaagcgctgcatgatgatggccagctccacctcgcttggcatgtaccccaaagagcgcatggccatgcccagctcctgcttggagatgaagccgttcccatcccggtccagaacccgaaaggcctctcggatttcatcgagctcctccacggagatattagccagctgttcgctgtcactgccagcagagagcgatcggttgaggtaattccccttgtacaacaagccggcggtcacatggtggaacggcatcttttccctcctgctgatctcgggggaaattctccaagatccatggctgggagttaaggagaatctctaagccatcaggaaggagcagggcactgcagctcctcagaat

SEQ ID NO: 9013 - RNA, 3446 nt, Homo sapiens
  source 1..3446: mol_type = other RNA
acgggttaggctcttgggagcttacatctgctccctcctccatattatggctgaagccttagttttacttgtgctcatcaggaatattcatagtctcccacagagggaaagtttctacagctgccctcaggctgttgccagtagcacttgcagaggtgaatgagaaaactttcattggagaccttgggtgctccaagtctgaaaaggcagtagggagaaagctgagcaggaagacagggagggagatcaggaacacacaacgcaccaaaaaatcctacccactgcatagagacaagaaagcttctggtggctcgctactggaaggggggaagcatgtagttttaggatgtaatcaaaagaagtaggagcaaggtaattccattacaaaataaagacctgagcttggaaaagtacaaagggaactattacatctagagattactggctaatctgactacacaagcttgaattcatagtagtggctgacatctaggaaaagtcaggaaattacagacttggaatggtgttgaaaacagatccttggattcagttctcttccccaacgaaaagtattctgcaggcaggagtaaattacctgttctgttggctaaactcataaacatcttttcccccaacctcctgaaaatgagtcagttgcagaatctgaaggccagaagatcttatgtgaaaatacagtcgtttgatctctccatctttccattttggattgcatttctctttttagctggggaagactaacaaagcaaactccaaggtaagggaaaggtaagatgcacaaggaccttaacttacaaaggtcatccggcatagagacgtggtgggtctccatgactccagatggctgggtgtgggtatcaaaacctcaccgccagtcccagtcccctcccccctcaacctgcctcacccctgccccaaagaagcagggatgagtgtgggagggaggacaagcttatattaggtgtaagcgattagggaagaatgacatcacacacgaagaagccaaatatatatatctgtctatgttatagagatgcccacgattatgcttctttttttctctaatggcagcacaggcggcaaagctgggagaaaggctctctgcaggttccaaaatgctggtgcgggatgggctctaggaacagaaagccaagtgccgacggaaactgagagcaccccagctctaccaatggcagtcctctagaaaaggcagtaagaacggaagcggtgaggggtgcagctgaagaccgccagggctgcaccccacttaatggctttcccctcatgccttgggggggtctccactgggtggaggaaggaagccagggtgggatggaaagccccctcttctgtggcaaccctgaagtcagcctcttggaactgagggttgacctcagcagagagtctcctgttgacccttgggttgaaagaatggggagtggaggtgactgtgtgttcatgcctctctcttgctctctcaccattatacctggatggctgctggaattccgagatgaagatgaagtttttctctagagttatgactgatggttgaagcaataatttggaaatcctggcgatttattgcattagaaaacaaaaccattaaagcactgaagacagccctttagtgtccctgccaaggagatgaagctgaagtgcaaccccagttgcactcaaccttgggttctttactgaacggttccatcgtccgcatccatccatagtccataggtccgtgtctgctgtgtggaggaagagtctgcccgcacggcatgcacatgcgcggtgagctgcaacacagtgtggctggcgggaggctgctactccatgccgctccggagtatctggttggctgcaatcagcatgacactgatgatgaaggccatagcaaaggcgcatatgaggctcttccggacgcaggtctgtctgttctgcttctgggaatgcactccttcaaactctgtttggcagttccccgaggtctcattcaggctctcttcctcattgataatgatgttctcaatgtccttcatcgttaggtggtctcggaaggcatgatagagaatgtgcttcaactcttccagagttatcctttgcatgtcaaactgccagaatatgctgtctatcgtgttcccaagaaaaccatcgcgaccttctgaagacaccagtttggggccaagaatggtcatgaattcatcaaaatccacctggccatccccgtccatgtccaagcgctgcatgatgatggccagctccacctcgcttggcatgtaccccaaagagcgcatggccatgcccagctcctgcttggagatgaagccgttcccatcccggtccagaacccgaaaggcctctcggatttcatcgagctcctccacggagatattagccagctgttcgctgtcactgccagcagagagcgatcggttgaggtaattccccttgtacaacaagccggcggtcacatggtggaacggcatcttttccctctgggtttccaagtactaagccgtgaccctgtgcaacatctctgtgacctggctacatctctgtttcttcatctgtaaaatgggagaaataaagcagatgacacctactaagcactaagctagtttgcctgctgagatggaatatgtgtttatgtgtatgcatataaaatgaatcatcagccacagatcagattaaaaagcagagcaactggttttccgaaccagcagtaggaatgctggaggctgagacgccacatcagtgttcagtacagatgtttgaggttttcttaccaggctataaaaatgtttacacagtaattaggcctgttatcagtacacaaacagattacaatttgcagaatgaatgaacagctcaaaaaccctctcggttttcatgaggttcggagcattttcctaattcttgggtttacaaaaataaattcggtttccaataacaaggagccacagctgagtgtaggggaaagggctctggggtgtgaaatgaactctgtttgacagtgcacatgtcactcagtctctctgactgagtctccccatctgtcaaatgagctaaccaaggttcctcttctcctttaaattccatggttctattactttgcagtcaatgtcttctaaacacatattcattcttttcaccacaaaaggatatgtttagttaatgatttttaaggtagtaattctgctgaatcacatgagactccaatccaacactattcagtcatattgagactgagtttgtggcagttaattcctgacaatgaagcccccaagcccagtctgtaggatgagaccacaaggtcaacttgggctttatgtgaacatccagctcttccagaacacatcaatggttctgagtaacacttgattgaggctgggtgcagtggctcacgcctgtaatcccagcactttgggagg

SEQ ID NO: 9014 - RNA, 3196 nt, Homo sapiens
  source 1..3196: mol_type = other RNA
acgggttaggctcttgggagcttacatctgctccctcctccatattatggctgaagccttagttttacttgtgctcatcaggaatattcatagtctcccacagagggaaagtttctacagctgccctcaggctgttgccagtagcacttgcagaggtgaatgagaaaactttcattggagaccttgggtgctccaagtctgaaaaggcagtagggagaaagctgagcaggaagacagggagggagatcaggaacacacaacgcaccaaaaaatcctacccactgcatagagacaagaaagcttctggtggctcgctactggaaggggggaagcatgtagttttaggatgtaatcaaaagaagtaggagcaaggtaattccattacaaaataaagacctgagcttggaaaagtacaaagggaactattacatctagagattactggctaatctgactacacaagcttgaattcatagtagtggctgacatctaggaaaagtcaggaaattacagacttggaatggtgttgaaaacagatccttggattcagttctcttccccaacgaaaagtattctgcaggcaggagtaaattacctgttctgttggctaaactcataaacatcttttcccccaacctcctgaaaatgagtcagttgcagaatctgaaggccagaagatcttatgtgaaaatacagtcgtttgatctctccatctttccattttggattgcatttctctttttagctggggaagactaacaaagcaaactccaaggtaagggaaaggtaagatgcacaaggaccttaacttacaaaggtcatccggcatagagacgtggtgggtctccatgactccagatggctgggtgtgggtatcaaaacctcaccgccagtcccagtcccctcccccctcaacctgcctcacccctgccccaaagaagcagggatgagtgtgggagggaggacaagcttatattaggtgtaagcgattagggaagaatgacatcacacacgaagaagccaaatatatatatctgtctatgttatagagatgcccacgattatgcttctttttttctctaatggcagcacaggcggcaaagctgggagaaaggctctctgcaggttccaaaatgctggtgcgggatgggctctaggaacagaaagccaagtgccgacggaaactgagagcaccccagctctaccaatggcagtcctctagaaaaggcagtaagaacggaagcggtgaggggtgcagctgaagaccgccagggctgcaccccacttaatggctttcccctcatgccttgggggggtctccactgggtggaggaaggaagccagggtgggatggaaagccccctcttctgtggcaaccctgaagtcagcctcttggaactgagggttgacctcagcagagagtctcctgttgacccttgggttgaaagaatggggagtggaggtgactgtgtgttcatgcctctctcttgctctctcaccattatacctggatggctgctggaattccgagatgaagatgaagtttttctctagagttatgactgatggttgaagcaataatttggaaatcctggcgatttattgcattagaaaacaaaaccattaaagcactgaagacagccctttagtgtccctgccaaggagatgaagctgaagtgcaaccccagttgcactcaaccttgggttctttactgaacggttccatcgtccgcatccatccatagtccataggtccgtgtctgctgtgtggaggaagagtctgcccgcacggcatgcacatgcgcggtgagctgcaacacagtgtggctggcgggaggctgctactccatgccgctccggagtatctggttggctgcaatcagcatgacactgatgatgaaggccatagcaaaggcgcatatgaggctcttccggacgcaggtctgtctgttctgcttctgggaatgcactccttcaaactctgtttggcagttccccgaggtctcattcaggctctcttcctcattgataatgatgttctcaatgtccttcatcgttaggtggtctcggaaggcatgatagagaatgtgcttcaactcttccagagttatcctttgcatgtcaaactgccagaatatgctgtctatcgtgttcccaagaaaaccatcgcgaccttctgaagacaccagtttggggccaagaatggtcatgaattcatcaaaatccacctggccatccccgtccatgtccaagcgctgcatgatgatggccagctccacctcgcttggcatgtaccccaaagagcgcatggccatgcccagctcctgcttggagatgaagccgttcccatcccggtccagaacccgaaaggcctctcggatttcatcgagctcctccacggagatattagccagctgttcgctgtcactgccagcagagagcgatcggttgaggtaattccccttgtacaacaagccggcggtcacatggtggaacggcatcttttccctcttgctgggccggggctccgcagcccggcagccgaggcgcctccgcacagcgcggggggcttcctccgaggcccgcagggagggggcggtgcggaatggatgcgccgagcgggcagcgctcagcctctcgctcacacccccagcaggcagccgcgtccccgtgccggcatcctcgctgccgccggctccctcggcgcccccgggccgctccccacgcgcgcgccgggacctgcacgagccccctcgtcgactcggagcgcgatctgggcgcgtgcctccctgtccttgtcctctgctctcgtctggggacgtgtgccccgcaccccctgcaccgcgcgctcctctacccctcccgctcccgctggccgcgcgggttcagcccatgtgcgcggctgcctcgctgcgccccggagcccagtggccgaggccccgctggagttgcgcgccctagaaactccatgcagctccggcctcctccccagctcctccccagcggatcccccagggccttgccgccgacagcaccacactcctcgctctgccggcgcccgcgttcaggagccgggcttctgggctcgccttggccgcctgcgccccagctcctccgagggtcggggagcccccaccccccaacctccgcctctccaatggctccctcggtttccaagcagcgcaacctgaggaac

SEQ ID NO: 9015 - RNA, 2782 nt, Homo sapiens
  source 1..2782: mol_type = other RNA
acgggttaggctcttgggagcttacatctgctccctcctccatattatggctgaagccttagttttacttgtgctcatcaggaatattcatagtctcccacagagggaaagtttctacagctgccctcaggctgttgccagtagcacttgcagaggtgaatgagaaaactttcattggagaccttgggtgctccaagtctgaaaaggcagtagggagaaagctgagcaggaagacagggagggagatcaggaacacacaacgcaccaaaaaatcctacccactgcatagagacaagaaagcttctggtggctcgctactggaaggggggaagcatgtagttttaggatgtaatcaaaagaagtaggagcaaggtaattccattacaaaataaagacctgagcttggaaaagtacaaagggaactattacatctagagattactggctaatctgactacacaagcttgaattcatagtagtggctgacatctaggaaaagtcaggaaattacagacttggaatggtgttgaaaacagatccttggattcagttctcttccccaacgaaaagtattctgcaggcaggagtaaattacctgttctgttggctaaactcataaacatcttttcccccaacctcctgaaaatgagtcagttgcagaatctgaaggccagaagatcttatgtgaaaatacagtcgtttgatctctccatctttccattttggattgcatttctctttttagctggggaagactaacaaagcaaactccaaggtaagggaaaggtaagatgcacaaggaccttaacttacaaaggtcatccggcatagagacgtggtgggtctccatgactccagatggctgggtgtgggtatcaaaacctcaccgccagtcccagtcccctcccccctcaacctgcctcacccctgccccaaagaagcagggatgagtgtgggagggaggacaagcttatattaggtgtaagcgattagggaagaatgacatcacacacgaagaagccaaatatatatatctgtctatgttatagagatgcccacgattatgcttctttttttctctaatggcagcacaggcggcaaagctgggagaaaggctctctgcaggttccaaaatgctggtgcgggatgggctctaggaacagaaagccaagtgccgacggaaactgagagcaccccagctctaccaatggcagtcctctagaaaaggcagtaagaacggaagcggtgaggggtgcagctgaagaccgccagggctgcaccccacttaatggctttcccctcatgccttgggggggtctccactgggtggaggaaggaagccagggtgggatggaaagccccctcttctgtggcaaccctgaagtcagcctcttggaactgagggttgacctcagcagagagtctcctgttgacccttgggttgaaagaatggggagtggaggtgactgtgtgttcatgcctctctcttgctctctcaccattatacctggatggctgctggaattccgagatgaagatgaagtttttctctagagttatgactgatggttgaagcaataatttggaaatcctggcgatttattgcattagaaaacaaaaccattaaagcactgaagacagccctttagtgtccctgccaaggagatgaagctgaagtgcaaccccagttgcactcaaccttgggttctttactgaacggttccatcgtccgcatccatccatagtccataggtccgtgtctgctgtgtggaggaagagtctgcccgcacggcatgcacatgcgcggtgagctgcaacacagtgtggctggcgggaggctgctactccatgccgctccggagtatctggttggctgcaatcagcatgacactgatgatgaaggccatagcaaaggcgcatatgaggctcttccggacgcaggtctgtctgttctgcttctgggaatgcactccttcaaactctgtttggcagttccccgaggtctcattcaggctctcttcctcattgataatgatgttctcaatgtccttcatcgttaggtggtctcggaaggcatgatagagaatgtgcttcaactcttccagagttatcctttgcatgtcaaactgccagaatatgctgtctatcgtgttcccaagaaaaccatcgcgaccttctgaagacaccagtttggggccaagaatggtcatgaattcatcaaaatccacctggccatccccgtccatgtccaagcgctgcatgatgatggccagctccacctcgcttggcatgtaccccaaagagcgcatggccatgcccagctcctgcttggagatgaagccgttcccatcccggtccagaacccgaaaggcctctcggatttcatcgagctcctccacggagatattagccagctgttcgctgtcactgccagcagagagcgatcggttgaggtaattccccttgtacaacaagccggcggtcacatggtggaacggcatcttttccctgctgctgcctaggcgccctcggaccaagtctcgggaagttcactccgcgctgcgctagtccggagaaactaggaacccgagtaaacccagactgtccggggaagacggatcccacccccacctgggcgccagacccatccagctgcttggagctcagagactaggtcccagccggactgcagaggcctctctggttaccccttgcaccctggcgcccccggactcggggtgggtggcggcgaggagcgtgcgcccagaaaggcaagcagtca

SEQ ID NO: 9016 - RNA, 3195 nt, Homo sapiens
  source 1..3195: mol_type = other RNA
acgggttaggctcttgggagcttacatctgctccctcctccatattatggctgaagccttagttttacttgtgctcatcaggaatattcatagtctcccacagagggaaagtttctacagctgccctcaggctgttgccagtagcacttgcagaggtgaatgagaaaactttcattggagaccttgggtgctccaagtctgaaaaggcagtagggagaaagctgagcaggaagacagggagggagatcaggaacacacaacgcaccaaaaaatcctacccactgcatagagacaagaaagcttctggtggctcgctactggaaggggggaagcatgtagttttaggatgtaatcaaaagaagtaggagcaaggtaattccattacaaaataaagacctgagcttggaaaagtacaaagggaactattacatctagagattactggctaatctgactacacaagcttgaattcatagtagtggctgacatctaggaaaagtcaggaaattacagacttggaatggtgttgaaaacagatccttggattcagttctcttccccaacgaaaagtattctgcaggcaggagtaaattacctgttctgttggctaaactcataaacatcttttcccccaacctcctgaaaatgagtcagttgcagaatctgaaggccagaagatcttatgtgaaaatacagtcgtttgatctctccatctttccattttggattgcatttctctttttagctggggaagactaacaaagcaaactccaaggtaagggaaaggtaagatgcacaaggaccttaacttacaaaggtcatccggcatagagacgtggtgggtctccatgactccagatggctgggtgtgggtatcaaaacctcaccgccagtcccagtcccctcccccctcaacctgcctcacccctgccccaaagaagcagggatgagtgtgggagggaggacaagcttatattaggtgtaagcgattagggaagaatgacatcacacacgaagaagccaaatatatatatctgtctatgttatagagatgcccacgattatgcttctttttttctctaatggcagcacaggcggcaaagctgggagaaaggctctctgcaggttccaaaatgctggtgcgggatgggctctaggaacagaaagccaagtgccgacggaaactgagagcaccccagctctaccaatggcagtcctctagaaaaggcagtaagaacggaagcggtgaggggtgcagctgaagaccgccagggctgcaccccacttaatggctttcccctcatgccttgggggggtctccactgggtggaggaaggaagccagggtgggatggaaagccccctcttctgtggcaaccctgaagtcagcctcttggaactgagggttgacctcagcagagagtctcctgttgacccttgggttgaaagaatggggagtggaggtgactgtgtgttcatgcctctctcttgctctctcaccattatacctggatggctgctggaattccgagatgaagatgaagtttttctctagagttatgactgatggttgaagcaataatttggaaatcctggcgatttattgcattagaaaacaaaaccattaaagcactgaagacagccctttagtgtccctgccaaggagatgaagctgaagtgcaaccccagttgcactcaaccttgggttctttactgaacggttccatcgtccgcatccatccatagtccataggtccgtgtctgctgtgtggaggaagagtctgcccgcacggcatgcacatgcgcggtgagctgcaacacagtgtggctggcgggaggctgctactccatgccgctccggagtatctggttggctgcaatcagcatgacactgatgatgaaggccatagcaaaggcgcatatgaggctcttccggacgcaggtctgtctgttctgcttctgggaatgcactccttcaaactctgtttggcagttccccgaggtctcattcaggctctcttcctcattgataatgatgttctcaatgtccttcatcgttaggtggtctcggaaggcatgatagagaatgtgcttcaactcttccagagttatcctttgcatgtcaaactgccagaatatgctgtctatcgtgttcccaagaaaaccatcgcgaccttctgaagacaccagtttggggccaagaatggtcatgaattcatcaaaatccacctggccatccccgtccatgtccaagcgctgcatgatgatggccagctccacctcgcttggcatgtaccccaaagagcgcatggccatgcccagctcctgcttggagatgaagccgttcccatcccggtccagaacccgaaaggcctctcggatttcatcgagctcctccacggagatattagccagctgttcgctgtcactgccagcagagagcgatcggttgaggtaattccccttgtacaacaagccggcggtcacatggtggaacggcatcttttccctggccaaagcaggctagtccttccttacagcaccctcctctcccgggtccccagtttcttgtcccctcttggtggcaaagactgctcaccagctcagatgtcttcaattcccagaaccagagaaaagatacatgtgaaaaatttcacaccaatcagaacaaaagcaggcaatgctgctctaagcctctcatgcaaacaactcagcaatcacctctccactgtttggttcaactgccagggaagtttgggcgtttttgtcagccagcagcacagtgtgtgtgtgtgtgtgtgtgtgtgtgtgtgtgtgtgtgtgtgtgtgtgtgtgtgtgtctcacctgggtgtggtttcagagtccctgaggcactcattgtgggtgccacgcctttagcatttagcatttcctaacctgtattattactatcttgtatagaccctacttccctagtaatcttttttaaatatgtttttgttatttttataggtacatggtaggtgtacatatttatggggtacatgagatgttttgttacaggcatgcaatgtgaaataagctcatcatggagaaccgggtagcattccctcaaacattcatcctttgagttacaaacagtccaattacactctaagttattgtaaaatatgagttattgactatagtcactgtgttgtgctatcaaataatagg

SEQ ID NO: 9017 - RNA, 2646 nt, Homo sapiens
  source 1..2646: mol_type = other RNA
acgggttaggctcttgggagcttacatctgctccctcctccatattatggctgaagccttagttttacttgtgctcatcaggaatattcatagtctcccacagagggaaagtttctacagctgccctcaggctgttgccagtagcacttgcagaggtgaatgagaaaactttcattggagaccttgggtgctccaagtctgaaaaggcagtagggagaaagctgagcaggaagacagggagggagatcaggaacacacaacgcaccaaaaaatcctacccactgcatagagacaagaaagcttctggtggctcgctactggaaggggggaagcatgtagttttaggatgtaatcaaaagaagtaggagcaaggtaattccattacaaaataaagacctgagcttggaaaagtacaaagggaactattacatctagagattactggctaatctgactacacaagcttgaattcatagtagtggctgacatctaggaaaagtcaggaaattacagacttggaatggtgttgaaaacagatccttggattcagttctcttccccaacgaaaagtattctgcaggcaggagtaaattacctgttctgttggctaaactcataaacatcttttcccccaacctcctgaaaatgagtcagttgcagaatctgaaggccagaagatcttatgtgaaaatacagtcgtttgatctctccatctttccattttggattgcatttctctttttagctggggaagactaacaaagcaaactccaaggtaagggaaaggtaagatgcacaaggaccttaacttacaaaggtcatccggcatagagacgtggtgggtctccatgactccagatggctgggtgtgggtatcaaaacctcaccgccagtcccagtcccctcccccctcaacctgcctcacccctgccccaaagaagcagggatgagtgtgggagggaggacaagcttatattaggtgtaagcgattagggaagaatgacatcacacacgaagaagccaaatatatatatctgtctatgttatagagatgcccacgattatgcttctttttttctctaatggcagcacaggcggcaaagctgggagaaaggctctctgcaggttccaaaatgctggtgcgggatgggctctaggaacagaaagccaagtgccgacggaaactgagagcaccccagctctaccaatggcagtcctctagaaaaggcagtaagaacggaagcggtgaggggtgcagctgaagaccgccagggctgcaccccacttaatggctttcccctcatgccttgggggggtctccactgggtggaggaaggaagccagggtgggatggaaagccccctcttctgtggcaaccctgaagtcagcctcttggaactgagggttgacctcagcagagagtctcctgttgacccttgggttgaaagaatggggagtggaggtgactgtgtgttcatgcctctctcttgctctctcaccattatacctggatggctgctggaattccgagatgaagatgaagtttttctctagagttatgactgatggttgaagcaataatttggaaatcctggcgatttattgcattagaaaacaaaaccattaaagcactgaagacagccctttagtgtccctgccaaggagatgaagctgaagtgcaaccccagttgcactcaaccttgggttctttactgaacggttccatcgtccgcatccatccatagtccataggtccgtgtctgctgtgtggaggaagagtctgcccgcacggcatgcacatgcgcggtgagctgcaacacagtgtggctggcgggaggctgctactccatgccgctccggagtatctggttggctgcaatcagcatgacactgatgatgaaggccatagcaaaggcgcatatgaggctcttccggacgcaggtctgtctgttctgcttctgggaatgcactccttcaaactctgtttggcagttccccgaggtctcattcaggctctcttcctcattgataatgatgttctcaatgtccttcatcgttaggtggtctcggaaggcatgatagagaatgtgcttcaactcttccagagttatcctttgcatgtcaaactgccagaatatgctgtctatcgtgttcccaagaaaaccatcgcgaccttctgaagacaccagtttggggccaagaatggtcatgaattcatcaaaatccacctggccatccccgtccatgtccaagcgctgcatgatgatggccagctccacctcgcttggcatgtaccccaaagagcgcatggccatgcccagctcctgcttggagatgaagccgttcccatcccggtccagaacccgaaaggcctctcggatttcatcgagctcctccacggagatattagccagctgttcgctgtcactgccagcagagagcgatcggttgaggtaattccccttgtacaacaagccggcggtcacatggtggaacggcatcttttccctgggctgcggtgcggctccgagtcccctgccctccctccccatcgcccgggcgcctgcgggcgggggcgcgcagcctggtggccactggcgcctgggggctagaagagcggctcccagcctccagcccgcacggtgc

SEQ ID NO: 9018 - RNA, 3130 nt, Homo sapiens
  source 1..3130: mol_type = other RNA
acgggttaggctcttgggagcttacatctgctccctcctccatattatggctgaagccttagttttacttgtgctcatcaggaatattcatagtctcccacagagggaaagtttctacagctgccctcaggctgttgccagtagcacttgcagaggtgaatgagaaaactttcattggagaccttgggtgctccaagtctgaaaaggcagtagggagaaagctgagcaggaagacagggagggagatcaggaacacacaacgcaccaaaaaatcctacccactgcatagagacaagaaagcttctggtggctcgctactggaaggggggaagcatgtagttttaggatgtaatcaaaagaagtaggagcaaggtaattccattacaaaataaagacctgagcttggaaaagtacaaagggaactattacatctagagattactggctaatctgactacacaagcttgaattcatagtagtggctgacatctaggaaaagtcaggaaattacagacttggaatggtgttgaaaacagatccttggattcagttctcttccccaacgaaaagtattctgcaggcaggagtaaattacctgttctgttggctaaactcataaacatcttttcccccaacctcctgaaaatgagtcagttgcagaatctgaaggccagaagatcttatgtgaaaatacagtcgtttgatctctccatctttccattttggattgcatttctctttttagctggggaagactaacaaagcaaactccaaggtaagggaaaggtaagatgcacaaggaccttaacttacaaaggtcatccggcatagagacgtggtgggtctccatgactccagatggctgggtgtgggtatcaaaacctcaccgccagtcccagtcccctcccccctcaacctgcctcacccctgccccaaagaagcagggatgagtgtgggagggaggacaagcttatattaggtgtaagcgattagggaagaatgacatcacacacgaagaagccaaatatatatatctgtctatgttatagagatgcccacgattatgcttctttttttctctaatggcagcacaggcggcaaagctgggagaaaggctctctgcaggttccaaaatgctggtgcgggatgggctctaggaacagaaagccaagtgccgacggaaactgagagcaccccagctctaccaatggcagtcctctagaaaaggcagtaagaacggaagcggtgaggggtgcagctgaagaccgccagggctgcaccccacttaatggctttcccctcatgccttgggggggtctccactgggtggaggaaggaagccagggtgggatggaaagccccctcttctgtggcaaccctgaagtcagcctcttggaactgagggttgacctcagcagagagtctcctgttgacccttgggttgaaagaatggggagtggaggtgactgtgtgttcatgcctctctcttgctctctcaccattatacctggatggctgctggaattccgagatgaagatgaagtttttctctagagttatgactgatggttgaagcaataatttggaaatcctggcgatttattgcattagaaaacaaaaccattaaagcactgaagacagccctttagtgtccctgccaaggagatgaagctgaagtgcaaccccagttgcactcaaccttgggttctttactgaacggttccatcgtccgcatccatccatagtccataggtccgtgtctgctgtgtggaggaagagtctgcccgcacggcatgcacatgcgcggtgagctgcaacacagtgtggctggcgggaggctgctactccatgccgctccggagtatctggttggctgcaatcagcatgacactgatgatgaaggccatagcaaaggcgcatatgaggctcttccggacgcaggtctgtctgttctgcttctgggaatgcactccttcaaactctgtttggcagttccccgaggtctcattcaggctctcttcctcattgataatgatgttctcaatgtccttcatcgttaggtggtctcggaaggcatgatagagaatgtgcttcaactcttccagagttatcctttgcatgtcaaactgccagaatatgctgtctatcgtgttcccaagaaaaccatcgcgaccttctgaagacaccagtttggggccaagaatggtcatgaattcatcaaaatccacctggccatccccgtccatgtccaagcgctgcatgatgatggccagctccacctcgcttggcatgtaccccaaagagcgcatggccatgcccagctcctgcttggagatgaagccgttcccatcccggtccagaacccgaaaggcctctcggatttcatcgagctcctccacggagatattagccagctgttcgctgtcactgccagcagagagcgatcggttgaggtaattccccttgtacaacaagccggcggtcacatggtggaacggcatcttttccctgtgtgcggaatttattccttctgctgggttgttggtctcgccgactttaagaataaaaccacggacctcgcggtgagtgttacagctcttaaagatggcgcgtccggagtcgtctgctcctcccggtgggcttgcggtcttgctgacttcaagaacgaagacgcagaccgcggccgtgagctttaaaggtggcgcggacccagagtaagcagtaagctcctgctgatctcgggggaaattctccaagatccatggctgggagttaaggagaatctctaagccatcaggaaggagcagggcactgcagctcctcagaatgatggaccggggcgagctttaattaacagggtctgatgcctcttcttttttggtaactgagcagatttaaagggctagagtcccaatttgaagggtgccagtgctgctgccgtggctgctgccgtgtctgctctggctgctgctcctgctgctgggaaagcttcctgcagccctctcactccagcaagaaaacggggctgagaaggtggaaaagtgcccccagaaacaccggagtctctcgggctgcatggtttgaatcggaaccacagggctgtggacccacgcactgcctaccctaggaa

SEQ ID NO: 9019 - RNA, 2817 nt, Homo sapiens
  source 1..2817: mol_type = other RNA
acgggttaggctcttgggagcttacatctgctccctcctccatattatggctgaagccttagttttacttgtgctcatcaggaatattcatagtctcccacagagggaaagtttctacagctgccctcaggctgttgccagtagcacttgcagaggtgaatgagaaaactttcattggagaccttgggtgctccaagtctgaaaaggcagtagggagaaagctgagcaggaagacagggagggagatcaggaacacacaacgcaccaaaaaatcctacccactgcatagagacaagaaagcttctggtggctcgctactggaaggggggaagcatgtagttttaggatgtaatcaaaagaagtaggagcaaggtaattccattacaaaataaagacctgagcttggaaaagtacaaagggaactattacatctagagattactggctaatctgactacacaagcttgaattcatagtagtggctgacatctaggaaaagtcaggaaattacagacttggaatggtgttgaaaacagatccttggattcagttctcttccccaacgaaaagtattctgcaggcaggagtaaattacctgttctgttggctaaactcataaacatcttttcccccaacctcctgaaaatgagtcagttgcagaatctgaaggccagaagatcttatgtgaaaatacagtcgtttgatctctccatctttccattttggattgcatttctctttttagctggggaagactaacaaagcaaactccaaggtaagggaaaggtaagatgcacaaggaccttaacttacaaaggtcatccggcatagagacgtggtgggtctccatgactccagatggctgggtgtgggtatcaaaacctcaccgccagtcccagtcccctcccccctcaacctgcctcacccctgccccaaagaagcagggatgagtgtgggagggaggacaagcttatattaggtgtaagcgattagggaagaatgacatcacacacgaagaagccaaatatatatatctgtctatgttatagagatgcccacgattatgcttctttttttctctaatggcagcacaggcggcaaagctgggagaaaggctctctgcaggttccaaaatgctggtgcgggatgggctctaggaacagaaagccaagtgccgacggaaactgagagcaccccagctctaccaatggcagtcctctagaaaaggcagtaagaacggaagcggtgaggggtgcagctgaagaccgccagggctgcaccccacttaatggctttcccctcatgccttgggggggtctccactgggtggaggaaggaagccagggtgggatggaaagccccctcttctgtggcaaccctgaagtcagcctcttggaactgagggttgacctcagcagagagtctcctgttgacccttgggttgaaagaatggggagtggaggtgactgtgtgttcatgcctctctcttgctctctcaccattatacctggatggctgctggaattccgagatgaagatgaagtttttctctagagttatgactgatggttgaagcaataatttggaaatcctggcgatttattgcattagaaaacaaaaccattaaagcactgaagacagccctttagtgtccctgccaaggagatgaagctgaagtgcaaccccagttgcactcaaccttgggttctttactgaacggttccatcgtccgcatccatccatagtccataggtccgtgtctgctgtgtggaggaagagtctgcccgcacggcatgcacatgcgcggtgagctgcaacacagtgtggctggcgggaggctgctactccatgccgctccggagtatctggttggctgcaatcagcatgacactgatgatgaaggccatagcaaaggcgcatatgaggctcttccggacgcaggtctgtctgttctgcttctgggaatgcactccttcaaactctgtttggcagttccccgaggtctcattcaggctctcttcctcattgataatgatgttctcaatgtccttcatcgttaggtggtctcggaaggcatgatagagaatgtgcttcaactcttccagagttatcctttgcatgtcaaactgccagaatatgctgtctatcgtgttcccaagaaaaccatcgcgaccttctgaagacaccagtttggggccaagaatggtcatgaattcatcaaaatccacctggccatccccgtccatgtccaagcgctgcatgatgatggccagctccacctcgcttggcatgtaccccaaagagcgcatggccatgcccagctcctgcttggagatgaagccgttcccatcccggtccagaacccgaaaggcctctcggatttcatcgagctcctccacggagatattagccagctgttcgctgtcactgccagcagagagcgatcggttgaggtaattccccttgtacaacaagccggcggtcacatggtggaacggcatcttttccctgtgtgcggaatttattccttctgctgggttgttggtctcgccgactttaagaataaaaccacggacctcgcggtgagtgttacagctcttaaagatggcgcgtccggagtcgtctgctcctcccggtgggcttgcggtcttgctgacttcaagaacgaagacgcagaccgcggccgtgagctttaaaggtggcgcggacccagagtaagcagtaagctttattaagaagcaggaaagaaaaaaacacaaactcaagcggatagcaccccagcgagcttccccagcgggctcggggagccagctttta

SEQ ID NO: 9020 - RNA, 3483 nt, Homo sapiens
  source 1..3483: mol_type = other RNA
acgggttaggctcttgggagcttacatctgctccctcctccatattatggctgaagccttagttttacttgtgctcatcaggaatattcatagtctcccacagagggaaagtttctacagctgccctcaggctgttgccagtagcacttgcagaggtgaatgagaaaactttcattggagaccttgggtgctccaagtctgaaaaggcagtagggagaaagctgagcaggaagacagggagggagatcaggaacacacaacgcaccaaaaaatcctacccactgcatagagacaagaaagcttctggtggctcgctactggaaggggggaagcatgtagttttaggatgtaatcaaaagaagtaggagcaaggtaattccattacaaaataaagacctgagcttggaaaagtacaaagggaactattacatctagagattactggctaatctgactacacaagcttgaattcatagtagtggctgacatctaggaaaagtcaggaaattacagacttggaatggtgttgaaaacagatccttggattcagttctcttccccaacgaaaagtattctgcaggcaggagtaaattacctgttctgttggctaaactcataaacatcttttcccccaacctcctgaaaatgagtcagttgcagaatctgaaggccagaagatcttatgtgaaaatacagtcgtttgatctctccatctttccattttggattgcatttctctttttagctggggaagactaacaaagcaaactccaaggtaagggaaaggtaagatgcacaaggaccttaacttacaaaggtcatccggcatagagacgtggtgggtctccatgactccagatggctgggtgtgggtatcaaaacctcaccgccagtcccagtcccctcccccctcaacctgcctcacccctgccccaaagaagcagggatgagtgtgggagggaggacaagcttatattaggtgtaagcgattagggaagaatgacatcacacacgaagaagccaaatatatatatctgtctatgttatagagatgcccacgattatgcttctttttttctctaatggcagcacaggcggcaaagctgggagaaaggctctctgcaggttccaaaatgctggtgcgggatgggctctaggaacagaaagccaagtgccgacggaaactgagagcaccccagctctaccaatggcagtcctctagaaaaggcagtaagaacggaagcggtgaggggtgcagctgaagaccgccagggctgcaccccacttaatggctttcccctcatgccttgggggggtctccactgggtggaggaaggaagccagggtgggatggaaagccccctcttctgtggcaaccctgaagtcagcctcttggaactgagggttgacctcagcagagagtctcctgttgacccttgggttgaaagaatggggagtggaggtgactgtgtgttcatgcctctctcttgctctctcaccattatacctggatggctgctggaattccgagatgaagatgaagtttttctctagagttatgactgatggttgaagcaataatttggaaatcctggcgatttattgcattagaaaacaaaaccattaaagcactgaagacagccctttagtgtccctgccaaggagatgaagctgaagtgcaaccccagttgcactcaaccttgggttctttactgaacggttccatcgtccgcatccatccatagtccataggtccgtgtctgctgtgtggaggaagagtctgcccgcacggcatgcacatgcgcggtgagctgcaacacagtgtggctggcgggaggctgctactccatgccgctccggagtatctggttggctgcaatcagcatgacactgatgatgaaggccatagcaaaggcgcatatgaggctcttccggacgcaggtctgtctgttctgcttctgggaatgcactccttcaaactctgtttggcagttccccgaggtctcattcaggctctcttcctcattgataatgatgttctcaatgtccttcatcgttaggtggtctcggaaggcatgatagagaatgtgcttcaactcttccagagttatcctttgcatgtcaaactgccagaatatgctgtctatcgtgttcccaagaaaaccatcgcgaccttctgaagacaccagtttggggccaagaatggtcatgaattcatcaaaatccacctggccatccccgtccatgtccaagcgctgcatgatgatggccagctccacctcgcttggcatgtaccccaaagagcgcatggccatgcccagctcctgcttggagatgaagccgttcccatcccggtccagaacccgaaaggcctctcggatttcatcgagctcctccacggagatattagccagctgttcgctgtcactgccagcagagagcgatcggttgaggtaattccccttgtacaacaagccggcggtcacatggtggaacggcatcttttcccttcaggtaattagatgaacgctcctgctggaagaaatcctgcaccagcttcacaaggatgccggcgctggcctgccgacaggaatgcttttggcaggtgattttgagttgttctttctgaaagtaattacacaaaaagttccactgcttgttaaggctccttcttaaggctgttttgatctcttttaattaataagttgaatatggaaggatttaattgtgatgaatttctatgtaacttccttcaagatccccacgtaaagtggtcctgctaagtccaccatacacttctagctgctcagacacctgtatcaaaccgagagccttagatagctttctgcaaagtttgagagaatcctgctggctgaggcctctcccaagacagtgagaggtcagggattatttgatctacgggaaataactgcacactgtacccaacattgattgttgagagttctctagaacagcacttttaagactttagtagcttagtttgctcaggttaccgtaacaaaagactacagaccgggtggcttaaacaacagaaattaattttcttatagcctgaaggctggatgtctaagatcaagaggtcaacatggtcaggttctgatgaggactctcttcctggcttacaaatggccaccttcttgctctgtcctcacatggtcggggagagacagaaagagggagagagggcaagctctctggtatctctacttataagggcactaaattccattatgagggacccaccctcaagacatcatctaaacttaattacctcctgaagactaaagttaccttgcccaaattcctatctaaggggtctagggagtcatgccctacaaaccataaacactcatcagatgggttttatctaaccttgtatatcatgacttactttccaaactgacactggtataacatgacaagacaaggaagaaaatcaaaaaattttaccccaaaacatgt

SEQ ID NO: 9021 - RNA, 62 nt, Homo sapiens
  source 1..62: mol_type = other RNA
actcaaaagatggcggcactttcaccagagagcagaaagtgcccccacagtttgagtgccac

SEQ ID NO: 9022 - RNA, 3627 nt, Homo sapiens
  source 1..3627: mol_type = other RNA
actcaaaagatggcggcactttctgagcaagtatctgaactggaccttttccaagggaagcagtccccgtggccacagactgccccctgggttgtgccagcagcactggatacagactccaaagacccggcatgaagtcttgccagagtatcctggggccactgactggtctttctgagcctccattttctccccttcacaatgcaaataactatttcttagacttgttataggtaaaacatggaataaacaaagaagaaaacacctgtggagtgcctggtgtccagtataggttttttttgtttgtttgggacacagtcgtgctccgtcatccaggctgaggtggttgcggcacaatcacggctcactgcaacctcggcctcttgagctcaggtgatcctcccaccttagcttcccgagtagctgggactacaggtgtgtgccattatgcctggctaatttttttttgttgggggagagggggatagagacagggttttcccatgttgtccaggctggtctcaaattcctgggctcaagtgatccttctgccttggcctcccaatgtgctgggattacaggtgtcagtatagatttttattatctgttttctcagtcttcaaagggtcccacgttaaatgctacaccatttcctaaactcatgctcacatccctggctggttctacaggccttccaccaggacctctggaaccacttcttatcatgtgctgggagtggcatctgatgtatggggagatgcaaattcccacatacccccttactggccctttgttggtcccgaatggccagaatacatagatgttcagtaccaaaattacacacttgtgaaaaaccaatttggcactgttctttccacctttactgttgctggaaacttgaaacccagaatacaattttacggttagaccctgcaaattgcagtttgtcatgtaatcttttacattttggtccatggacttatgaataggatgccaaactctagttgactatgtatatgattactttttctttctacttaagcacaaaattcattattaagtggggaaatacaaagataatctcagattagtttacaaaagcaggcaaacaatgcatagctataattgcatatatacatataaaatgtatatataatatataatacacgggggtggagatagagaaggagagaggatatgacatcaagctattaactatactgatatgtagaaagcaaacaacttgatagtcaactcttactttatcacatctcatcagccccaaatatctcagagacttgctgctctgtgcaatcagggtggctccttggtctgtgatttctttacaccatccgacatccacagtctctattgtcatgctgtatcgcccaatggctatcagtgcataatctgtgattttacaggacaccaaatatagctctttcaggttttgtccttcctttgcaatgacctccacacacctgtcatttatgatccagttcagacagagattgagagagctaagatttttgcacctcttgacaatttccatcacggtttcattatccagttcagtgatatgacgtaggtccaagctggaaaggtttcttagcttggttaggtgaatgactcctttagaagtgactgaacaacccatgaagcctacatattgaagctcaggacagtgttcagcaaatgctttcactgactgatctgtcactaatttgttttcctgcatgtatatcctttgtaatttcagacagcccttagctatgacgatcatgccttcatctgagatcttgtaacactggccgaaatgaatatctttgagttctctgcattttgagcccagctgcttgagtccttcatcagtgagtttgtcctggttgcctacatgcactttctgaagtaaaggacagtgagaggcaaccgcaataatagaggtgtcagaaagctgtttacacctgtaggctgtatacctaagaagtccaggacatttaaatgctaaaacacatacgccattatcagacatactgcgacaatcagaaatgttgatttcaattatattctgacttcttgatgcaattttttccaacaattcatcagtgacctgctgacgactactaagatccagctgcttccaaaactggaagtctaaacaaaggtcacgccagtacttgcaaaccaatgatgcggaaaggcaacgctcatccagtgacaaattggaaaatatcttgagcaggatggacggcggcagctggttgatgtctggggtttcggggggcggctccctgtgacagtcgcaggggttttcgggggactcccgacagtccgcgtcgccacattcatgctgctgctgggcggacaagggggcggtgcccccggctcggacagcgtccccgccagcttcggtgggggcaccttcggaggtgggagaagagggcggagggcagagcggctgcgggggctgctccggggcctggcagcagccggcgtcggggggccggggcggcgaagcgcctccccccgcaggccctcccccgccaccgccgccgccgccgccgccgcagcccccgccgccgcagcggggctgcttgcagggggtgcaggcggggaccccggcccccttccgcttgcacaccatttcggggggcgtagggagctcggccggtgacggtgtcggcccccggaagagctgcacggcggcgggcggccccaggaagcgcaccggccccaagctggccaggaagagacttcggccctgctgctcccaggcggcggccgcagccagccccaactctttgcagcaggaggcgggcgacgaagccgaggcggcagcggcggcggcggcggcggccgaggatagcaggaagcggcgggcagcagcggcgcagtcctcggcggccagggccgcgtagcgccgcgccaggtgctgagaggaggaggcggcagcgtaggccccgtcccgcggcggcggcgagagcggcggctcctcctctgggccggcgggggcgggcgcgccgggactgtgcacgatgaagcagagcatgcagggcccgcggaagaagcagtcccggctccggggcgccgccggctgagggggcaccttggctggggtccggcggggcagcctgaggagagggcgccggcggcggcaccaactgcaacagcgaggcctcttctggctcgggcggttacgcggctccttcgagagaaggtggcccatatagaaggccccgaggagggggaccgggacgggagggagggagacccagagaggcgggctcccggcagcggggcaggccgctcgctggctcggcccccggaggggtcgcccttcctgcgcacacacacgcacacacgggcacacacgcgacggtggggggtgggcgtcagctgcgggccgccggagtgcccgacgggggctacatgctttgcccagggaagccgggagaacgatgggcgcgagctttggggacgcgagggagggagcgagcgagcctgccggctaggcgaccagtccgggcccggccagccggctcagtcagtcagcggagcggccggggaaaggccgggtcccgctcggaccattttaactgcggatccgccgccggcgcgcgcacccgc

SEQ ID NO: 9023 - RNA, 63 nt, Homo sapiens
  source 1..63: mol_type = other RNA
actcaaactgtgggggcactttctgctctctggtgaaagtgccgccatcttttgagtgttacc

SEQ ID NO: 9024 - RNA, 1931 nt, Homo sapiens
  source 1..1931: mol_type = other RNA
actcattctcctctgtccagcctgttctcctggggctttgctgctggagcctggatggggcgggtgggtcatcagggcagtgagccagacagaaagccccccgacctgtcagcctcttcagcctcctcagcctcctccactgccaccaccaggcctgaggtgggcaaggaacagggcacacaggctgggggcaggggctgggcggggggtggtggcgacagggccccctttagggccgggacagtgtcgtatatactggctgctcccagtgtgtggggctgtgggactggggccctgaggggctggggtcagagatggccgtgtagaggggccgctgcgagggccccatataggagaaggccgagtagaggccagaggcctggcccgagtggccataatagggtcctgagggctgatggtcagagtagtcaaactgggggcgggagatggaggggaaggctgagccatagtggggcaggctgagggaggtgtaggcgatctgtgaggtggatggctggtcggtgtagtgtgggggcccctggggccccgcggtctctgtcttcacctgggctttggcatccacaccaggtggtgagaccgtgggcagagccacgcctggtggcttggagatccaggcggagtgtccactggccacggccagggcactgcccagcccatagccggctgctgagtagctgctcacatggcctgggtgcccattgggcggcaggtactggtccaactcagccacatcaaaggtctccatgttggacattacctcgtggctgatctcaccaatgtccacgttgccgaagtcgatgtgaggcttcccgccctcccccatggagcgcccgtcccgcttcgggtctgccttgcccgactgcagctctgtcttcggggtggttggaggggtgggtgggccatggctctggcctgaggggtgctcggggttcccatctgacatgggggagccctctcctgggtgccggtggtccaagtgggcgctcttgtagtgggcctggatggcggcggtcccaccttgctcggcctccccaccggggcactccgcctcgccctgggcggccttcccgttcttccgccgcctgggctggtacttgtagtccgggtggtctttcttgtgctgcatacggagccgctcagcctcctcgatgaaggggcgcttgtcactttcgttcagcagcctccagagcttgcccagcgtcttgctgagctcagcgttgtgcaggtgcgggtactggtccgcgagcttcctgcgcgctgcctgagcccacaccatgaaggcgttcatgggccgcttgacgtgcggcttgcttttgctggcgccgttgacgcgcacgggcatgggcaccagcgtccagtcgtagccgctgagcacctggctgacggcctcgcggatgcacacggggaacttgtcatcgtccgcctcgccgtcctgctgctccttcttgaccttgcccagctcgcctggccccgggctggctcgcaggcccgatccgccgccgccgccgtcgggccctagcgagggcgcgctccccggggacaggcagcggggctcctccgagcccacggggctcagctccacctccgataggtcctgctcctccgccatgtcgcccccggccgccgccgccgccgcctcggccgcctcccccgggccagccgccggggtcctcgcaaagagtccaacgcccacctcctcggacctctcctccagtctggggctcgtccttaggaagtggaaaaccgtgtcccaaggtgtgcggtccagctcggggctgggaggtgacgctggtgggctgggagggaggggcggggggccctgagcctcaggccacggcctcgttaggacggagcctgaatccttaccaccaaccaccctggccggacagcccgagactgactgagcgact

SEQ ID NO: 9025 - RNA, 1245 nt, Homo sapiens
  source 1..1245: mol_type = other RNA
actcattctcctctgtccagtctgggaaaatgacatggacagctatcaagtctttcaagtgtactccaaggatggggattttgaagccatcgcagtcggcaaaggccttgcggtaattgcagtaattgccgttggaggagaccaactctgtcatttcattccagttctttgtaacttctgaagaaagatgagaatgggtctctttgaggcgtgaaatggaactatgactgaggcctcccaccactgccatcagggtgttaaaatttttgagctgaaggagcttctttgcaacattgataaactttgtgatgacttctgccctttgctggggggttggtttgctaagaaccatcaactggacccacttagagattccattaaataaagcaatcgatctttccaaggttggattattctccaggcagccatggatgacatagctttggtaatcagtgaatgagatccttctaaaagatttatgctccagaaaagtgaggtgctcagccaattcaatgggctccagatggtcaaacagcagacaggcttttcccttcttggatacttttttcctctgtgtgactcttctcatccagtcataggaaggaatgctggatatgtcgatgaggctgacgtgtttttcatatcctagttgactagctacttcccgaaattcctcagtcatacgaatcaaaccaagatccaaattaaactctgcaggaaacttcagaatccagtacctcatgaagtagcagatctttaatcgaaattcattgcagctttctccagtggcatttcgatacatgcagagaagtttttctgccaattcagtggaagataaataccatcggtgcatcagtagaactattcttggcaaataactattatccagctctccattgtcatcaaacatctcaatgcaagtgcacagcagttcatctaatgttgctgctttcccaaggccacttgatcccatggttatttagccgttgtcaaaaaactagagacattttcagcatcagatagaccatctccataatcatgcaagtcagcgatgttagtgcctagtggtgacctgtccttagttgtacttcaagaaaactccaaaaccatgcaattattaaggcctagagtcaggactccactataaaataaagcttctgtgttccctttcttcttattacttctacaagcatggatatcacaaaccatcatagttttgcctgctaatctagtgtaaagggtatc

SEQ ID NO: 9026 - RNA, 1654 nt, Homo sapiens
  source 1..1654: mol_type = other RNA
actcattctcctctgtccagtctgggaaaatgacatggacagctatcaagtctttcaagtgtactccaaggatggggattttgaagccatcgcagtcggcaaaggccttgcggtaattgcagtaattgccgttggaggagaccaactctgtcatttcattccagttctttgtaacttctgaagaaagatgagaatgggtctctttgaggcgtgaaatggaactatgactgaggcctcccaccactgccatcagggtgttaaaatttttgagctgaaggagcttctttgcaacattgataaactttgtgatgacttctgccctttgctggggggttggtttgctaagaaccatcaactggacccacttagagattccattaaataaagcaatcgatctttccaaggttggattattctccaggcagccatggatgacatagctttggtaatcagtgaatgagatccttctaaaagatttatgctccagaaaagtgaggtgctcagccaattcaatgggctccagatggtcaaacagcagacaggcttttcccttcttggatacttttttcctctgtgtgactcttctcatccagtcataggaaggaatgctggatatgtcgatgaggctgacgtgtttttcatatcctagttgactagctacttcccgaaattcctcagtcatacgaatcaaaccaagatccaaattaaactctgcaggaaacttcagaatccagtacctcatgaagtagcagatctttaatcgaaattcattgcagctttctccagtggcatttcgatacatgcagagaagtttttctgccaattcagtggaagataaataccatcggtgcatcagtagaactattcttggcaaataactattatccagctctccattgtcatcaaacatctcaatgcaagtgcacagcagttcatctaatgttgctgctttcccaaggccacttgatcccatggttatttagccgttgtcaaaaaactagagacattttcagcatcagatagaccatctccataatcatgcaagtcagcgatgttagtgcctagtggtgacctgtccttagttgtacttcaagaaaactctgttgtttccatacagatacagttccaaatctgaaagaattttaagggcagctagcatcattgggaaatgcatggaagaagcagtctgtagaactggtttattcaacctgaatgataagtattttggagaacctattttactaaatggatgattgtgtctaggaggatgcatgcctcttattaatagcttgaaagaaaattcaaagaggccccttggttctggtagacaacctgcccagtgaaatgaacacctaaagaagaggtacacactcagcatgatggcacatcattcttctggatgacctttatacttcaccctgtcactgcagactcatgaagcctgggcagagcgagccaggcgtggtactactggctgacctacttcggtgcaccaaggctcccatacatgtccccagaacatttgctcactagaatgttcccctccccatcctgatgcctccatggatcggtaagcatgagcacagctacattacgggccagggcagcttccagggtagaggcctgtcttaacaagctggtataacaaaacacc

SEQ ID NO: 9027 - RNA, 2950 nt, Homo sapiens
  source 1..2950: mol_type = other RNA
actcattctcctctgtccagtctgggaaaatgacatggacagctatcaagtctttcaagtgtactccaaggatggggattttgaagccatcgcagtcggcaaaggccttgcggtaattgcagtaattgccgttggaggagaccaactctgtcatttcattccagttctttgtaacttctgaagaaagatgagaatgggtctctttgaggcgtgaaatggaactatgactgaggcctcccaccactgccatcagggtgttaaaatttttgagctgaaggagcttctttgcaacattgataaactttgtgatgacttctgccctttgctggggggttggtttgctaagaaccatcaactggacccacttagagattccattaaataaagcaatcgatctttccaaggttggattattctccaggcagccatggatgacatagctttggtaatcagtgaatgagatccttctaaaagatttatgctccagaaaagtgaggtgctcagccaattcaatgggctccagatggtcaaacagcagacaggcttttcccttcttggatacttttttcctctgtgtgactcttctcatccagtcataggaaggaatgctggatatgtcgatgaggctgacgtgtttttcatatcctagttgactagctacttcccgaaattcctcagtcatacgaatcaaaccaagatccaaattaaactctgcaggaaacttcagaatccagtacctcatgaagtagcagatctttaatcgaaattcattgcagctttctccagtggcatttcgatacatgcagagaagtttttctgccaattcagtggaagataaataccatcggtgcatcagtagaactattcttggcaaataactattatccagctctccattgtcatcaaacatctcaatgcaagtgcacagcagttcatctaatgttgctgctttcccaaggccacttgatcccatggttatttagccgttgtcaaaaaactagagacattttcagcatcagatagaccatctccataatcatgcaagtcagcgatgttagtgcctagtggtgacctgtccttagttgtacttcaagaaaactctgttgtttccatacagatacagttccaaatctgaaagaattttaagggcagctagcatcattgggaaatgcatggaagaagcagtctgtagaactggtttattcaacctgaatgataagtattttggagaacctccacaggaataaaggtgctatactcaggcagaactttcaagaatgccgatggttttgttgggcaaggagcgtgcacactgaagagcagactgcagttttcatacctcaggaaacaaccaaattgtctctaaaaggtaacgttacatcatgccatagttggtataactccaacttgactatatgagtcttcaagacagaaaaatgatcactaagttcctttaaaaacattaccctaagctgcggcccggcacggtggctcacgcctctaatccaagcactttgggaggcccaggcgggcagatcacgaggtcaggaaatcgagaccatcctggctaacacagtgaaaccctgtctctactaaaaatacaaaaaaattagcccggcatggtggcgggcgcctatagtcccagctactcgggaggctgaggcaggagaatggcatgaacctgggaggcggagcttgcagtgagccgagattgtgccactgcactccagcctgggcgacaaagcgagactccatctcaaaaaaaaaaaaaatattaccctaagctagccaggcacagtggctcatgcctataatcccagcactttgggaagccaaggtgggtggatcacctgaggtcaggagttcgagaccagcctggccaacatggtgaaaacccatctctactaaaaacacaaaaattagctgggtgtggtggtgcacgcctgtagtcccagctactcaggaggctgaggcaagagaatcgcttgaacctgggaggcagaggttgcagtgagccaagattgtgccactgcactccagcttgggtgacagagtgggactctgtctgaaaaaacaaacaaacaaaattatcctaagcaaatacggtgtctgaagactaagctgaccctgtttccaaagtcaaatgtccataggctttggaaatatcatgagtggcatgtcgcaaatcggttatccagtcactctttgcctatctgaagagaatacaaattacacaactttttatcaccaaagataattccacagattgtgtaagtgcatggtcatgaaatagttgaaattggtctttctttgaaagatagcataactaggccaggcgcagtggctcatgcctgtaatcccagcactttgggaggccgaggtgggtggatcaccaggtcaggagatcgagaccatcctgctaacatgatgaaaccccgtctctattaaaaatacaaaaaaattagccaggcgtggtggtgggcacctgtagtcccagctactcgggaggctgaggcagaagaatggtgtgaacccgggaggcggagcttgcagtgagccgagatcgtgccactgcactccagcctgggcgacagagtgaaactccattgagaatcttggcagtgaaatcagagaatccaaatgggtcatcagaggggtgccgcaggttcaggtagattgggtgtagtttccatggcaaagaagagatatggatgttttaaaagaaaatatcctttgcagaactgcaataatgttgatccctatagtgaattgtctttttctttccacttcatcacctctagcaagtttctcttcaacgtgcctaaacacctagaattcctgttctgtcttctaaaatgctgtcatcacctccattgcccaaatctagttcaaaagtgaggagagaaaaaaaattgaaatttgcaagctgtttatgcctaacaacaacatt

SEQ ID NO: 9028 - RNA, 1414 nt, Homo sapiens
  source 1..1414: mol_type = other RNA
actcattctcctctgtccagtctgggaaaatgacatggacagctatcaagtctttcaagtgtactccaaggatggggattttgaagccatcgcagtcggcaaaggccttgcggtaattgcagtaattgccgttggaggagaccaactctgtcatttcattccagttctttgtaacttctgaagaaagatgagaatgggtctctttgaggcgtgaaatggaactatgactgaggcctcccaccactgccatcagggtgttaaaatttttgagctgaaggagcttctttgcaacattgataaactttgtgatgacttctgccctttgctggggggttggtttgctaagaaccatcaactggacccacttagagattccattaaataaagcaatcgatctttccaaggttggattattctccaggcagccatggatgacatagctttggtaatcagtgaatgagatccttctaaaagatttatgctccagaaaagtgaggtgctcagccaattcaatgggctccagatggtcaaacagcagacaggcttttcccttcttggatacttttttcctctgtgtgactcttctcatccagtcataggaaggaatgctggatatgtcgatgaggctgacgtgtttttcatatcctagttgactagctacttcccgaaattcctcagtcatacgaatcaaaccaagatccaaattaaactctgcaggaaacttcagaatccagtacctcatgaagtagcagatctttaatcgaaattcattgcagctttctccagtggcatttcgatacatgcagagaagtttttctgccaattcagtggaagataaataccatcggtgcatcagtagaactattcttggcaaataactattatccagctctccattgtcatcaaacatctcaatgcaagtgcacagcagttcatctaatgttgctgctttcccaaggccacttgatcccatggttatttagccgttgtcaaaaaactagagacattttcagcatcagatagaccatctccataatcatgcaagtcagcgatgttagtgcctagtggtgacctgtccttagttgtacttcaagaaaactctgttgtttccatacagatacagttccaaatctgaaagaattttaagggcagctagcatcattgggaaatgcatggaagaagcagtctgtagaactggtttattcaacctgaatgataagtattttggagaacctgtagtcccagctactcgggaggctgaggcagaagaatggtgtgaacccgggaggcggagcttgcagtgagccgagatcgtgccactgcactccagcctgggcgacagagtgaaactccattagggtggttttgtcgtggtatttttcacatcagcactctgcctgtccagctgccaagt

SEQ ID NO: 9029 - RNA, 1723 nt, Homo sapiens
  source 1..1723: mol_type = other RNA
actcattctcctctgtccagtctgggaaaatgacatggacagctatcaagtctttcaagtgtactccaaggatggggattttgaagccatcgcagtcggcaaaggccttgcggtaattgcagtaattgccgttggaggagaccaactctgtcatttcattccagttctttgtaacttctgaagaaagatgagaatgggtctctttgaggcgtgaaatggaactatgactgaggcctcccaccactgccatcagggtgttaaaatttttgagctgaaggagcttctttgcaacattgataaactttgtgatgacttctgccctttgctggggggttggtttgctaagaaccatcaactggacccacttagagattccattaaataaagcaatcgatctttccaaggttggattattctccaggcagccatggatgacatagctttggtaatcagtgaatgagatccttctaaaagatttatgctccagaaaagtgaggtgctcagccaattcaatgggctccagatggtcaaacagcagacaggcttttcccttcttggatacttttttcctctgtgtgactcttctcatccagtcataggaaggaatgctggatatgtcgatgaggctgacgtgtttttcatatcctagttgactagctacttcccgaaattcctcagtcatacgaatcaaaccaagatccaaattaaactctgcaggaaacttcagaatccagtacctcatgaagtagcagatctttaatcgaaattcattgcagctttctccagtggcatttcgatacatgcagagaagtttttctgccaattcagtggaagataaataccatcggtgcatcagtagaactattcttggcaaataactattatccagctctccattgtcatcaaacatctcaatgcaagtgcacagcagttcatctaatgttgctgctttcccaaggccacttgatcccatggttatttagccgttgtcaaaaaactagagacattttcagcatcagatagaccatctccataatcatgcaagtcagcgatgttagtgcctagtggtgacctgtccttagttgtacttcaagaaaactctgttgtttccatacagatacagttccaaatctgaaagaattttaagggcagctagcatcattgggaaatgcatggaagaagcagtctgtagaactggtttattcaacctgaatgataagtattttggagaacctgtagtcccagctactcgggaggctgaggcagaagaatggtgtgaacccgggaggcggagcttgcagtgagccgagatcgtgccactgcactccagcctgggcgacagagtgaaactccattgagaatcttggcagtgaaatcagagaatccaaatgggtcatcagaggggtgccgcaggttcaggtagattgggtgtagtttccatggcaaagaagagatatggatgttttaaaagaaaatatcctttgcagaactgcaataatgttgatccctatagtgaattgtctttttctttccacttcatcacctctagcaagtttctcttcaacgtgcctaaacacctagaattcctgttctgtcttctaaaatgctgtcatcacctccattgcccaaatctagttcaaaagtgaggagagaaaaaaaattgaaatttgcaagctgtttatgcctaacaacaacattgaagctgctaagctttgagctcaat

SEQ ID NO: 9030 - RNA, 1292 nt, Homo sapiens
  source 1..1292: mol_type = other RNA
actcattctcctctgtccagtctgggaaaatgacatggacagctatcaagtctttcaagtgtactccaaggatggggattttgaagccatcgcagtcggcaaaggccttgcggtaattgcagtaattgccgttggaggagaccaactctgtcatttcattccagttctttgtaacttctgaagaaagatgagaatgggtctctttgaggcgtgaaatggaactatgactgaggcctcccaccactgccatcagggtgttaaaatttttgagctgaaggagcttctttgcaacattgataaactttgtgatgacttctgccctttgctggggggttggtttgctaagaaccatcaactggacccacttagagattccattaaataaagcaatcgatctttccaaggttggattattctccaggcagccatggatgacatagctttggtaatcagtgaatgagatccttctaaaagatttatgctccagaaaagtgaggtgctcagccaattcaatgggctccagatggtcaaacagcagacaggcttttcccttcttggatacttttttcctctgtgtgactcttctcatccagtcataggaaggaatgctggatatgtcgatgaggctgacgtgtttttcatatcctagttgactagctacttcccgaaattcctcagtcatacgaatcaaaccaagatccaaattaaactctgcaggaaacttcagaatccagtacctcatgaagtagcagatctttaatcgaaattcattgcagctttctccagtggcatttcgatacatgcagagaagtttttctgccaattcagtggaagataaataccatcggtgcatcagtagaactattcttggcaaataactattatccagctctccattgtcatcaaacatctcaatgcaagtgcacagcagttcatctaatgttgctgctttcccaaggccacttgatcccatggttatttagccgttgtcaaaaaactagagacattttcagcatcagatagaccatctccataatcatgcaagtcagcgatgttagtgcctagtggtgacctgtccttagttgtacttcaagaaaactctgttgtttccatacagatacagttccaaatctgaaagaattttaagggcagctagcatcattgggaaatgcatggaagaagcagtctgtagaactggtttattcaacctgaatgataagtattttggagaactagggtggttttgtcgtggtatttttcacatcagcactctgcctgtccagctgccaagt

SEQ ID NO: 9031 - RNA, 1713 nt, Homo sapiens
  source 1..1713: mol_type = other RNA
actcattctcctctgtccagtctgggaaaatgacatggacagctatcaagtctttcaagtgtactccaaggatggggattttgaagccatcgcagtcggcaaaggccttgcggtaattgcagtaattgccgttggaggagaccaactctgtcatttcattccagttctttgtaacttctgaagaaagatgagaatgggtctctttgaggcgtgaaatggaactatgactgaggcctcccaccactgccatcagggtgttaaaatttttgagctgaaggagcttctttgcaacattgataaactttgtgatgacttctgccctttgctggggggttggtttgctaagaaccatcaactggacccacttagagattccattaaataaagcaatcgatctttccaaggttggattattctccaggcagccatggatgacatagctttggtaatcagtgaatgagatccttctaaaagatttatgctccagaaaagtgaggtgctcagccaattcaatgggctccagatggtcaaacagcagacaggcttttcccttcttggatacttttttcctctgtgtgactcttctcatccagtcataggaaggaatgctggatatgtcgatgaggctgacgtgtttttcatatcctagttgactagctacttcccgaaattcctcagtcatacgaatcaaaccaagatccaaattaaactctgcaggaaacttcagaatccagtacctcatgaagtagcagatctttaatcgaaattcattgcagctttctccagtggcatttcgatacatgcagagaagtttttctgccaattcagtggaagataaataccatcggtgcatcagtagaactattcttggcaaataactattatccagctctccattgtcatcaaacatctcaatgcaagtgcacagcagttcatctaatgttgctgctttcccaaggccacttgatcccatggttatttagccgttgtcaaaaaactagagacattttcagcatcagatagaccatctccataatcatgcaagtcagcgatgttagtgcctagtggtgacctgtccttagttgtacttcaagaaaactctgttgtttccatacagatacagttccaaatctgaaagaattttaagggcagctagcatcattgggaaatgcatggaagaagcagtctgtagaactggtttattcaacctgaatgataagtattttggagaactagggtggttttgtcgtggtatttttcacatcagcactctgcctgtccagctgccaagtgccggagcacgccgagagcagctgtttccttcaagctggggctctgagtcttaaccagtcacatgtacctcctgataaataccgcccgccaccgtgccaggaggtcagaaactgaagatcattcttctcctcactcgcaaaccacctcataacccctgagttggctcagccatctcatgagcatgcagagcgggatattccacaatttgttttcctttagtgacaaaagccaaacagctgataagtcacactgaagggcaggtcactgcaagtggaaagttaaatgtgtttgcgtgtgtgtgtgcgcagagggggagactggcaggctccatgctctctcatctcactcaagtttcactggggctctcgaacggcaagagagaggatcaccaactcgcacagcaggtggaagttgctctgt

SEQ ID NO: 9032 - RNA, 1601 nt, Homo sapiens
  source 1..1601: mol_type = other RNA
actcattctcctctgtccagtctgggaaaatgacatggacagctatcaagtctttcaagtgtactccaaggatggggattttgaagccatcgcagtcggcaaaggccttgcggtaattgcagtaattgccgttggaggagaccaactctgtcatttcattccagttctttgtaacttctgaagaaagatgagaatgggtctctttgaggcgtgaaatggaactatgactgaggcctcccaccactgccatcagggtgttaaaatttttgagctgaaggagcttctttgcaacattgataaactttgtgatgacttctgccctttgctggggggttggtttgctaagaaccatcaactggacccacttagagattccattaaataaagcaatcgatctttccaaggttggattattctccaggcagccatggatgacatagctttggtaatcagtgaatgagatccttctaaaagatttatgctccagaaaagtgaggtgctcagccaattcaatgggctccagatggtcaaacagcagacaggcttttcccttcttggatacttttttcctctgtgtgactcttctcatccagtcataggaaggaatgctggatatgtcgatgaggctgacgtgtttttcatatcctagttgactagctacttcccgaaattcctcagtcatacgaatcaaaccaagatccaaattaaactctgcaggaaacttcagaatccagtacctcatgaagtagcagatctttaatcgaaattcattgcagctttctccagtggcatttcgatacatgcagagaagtttttctgccaattcagtggaagataaataccatcggtgcatcagtagaactattcttggcaaataactattatccagctctccattgtcatcaaacatctcaatgcaagtgcacagcagttcatctaatgttgctgctttcccaaggccacttgatcccatggttatttagccgttgtcaaaaaactagagacattttcagcatcagatagaccatctccataatcatgcaagtcagcgatgttagtgcctagtggtgacctgtccttagttgtacttcaagaaaactctgttgtttccatacagatacagttccaaatctgaaagaattttaagggcagctagcatcattgggaaatgcatggaagaagcagtctgtagaactggtttattcaacctgaatgataagtattttggagaactgagaatcttggcagtgaaatcagagaatccaaatgggtcatcagaggggtgccgcaggttcaggtagattgggtgtagtttccatggcaaagaagagatatggatgttttaaaagaaaatatcctttgcagaactgcaataatgttgatccctatagtgaattgtctttttctttccacttcatcacctctagcaagtttctcttcaacgtgcctaaacacctagaattcctgttctgtcttctaaaatgctgtcatcacctccattgcccaaatctagttcaaaagtgaggagagaaaaaaaattgaaatttgcaagctgtttatgcctaacaacaacattgaagctgctaagctttgagctcaat

SEQ ID NO: 9033 - RNA, 1309 nt, Homo sapiens
  source 1..1309: mol_type = other RNA
actcattctcctctgtccagtctgggaaaatgacatggacagctatcaagtctttcaagtgtactccaaggatggggattttgaagccatcgcagtcggcaaaggccttgcggtaattgcagtaattgccgttggaggagaccaactctgtcatttcattccagttctttgtaacttctgaagaaagatgagaatgggtctctttgaggcgtgaaatggaactatgactgaggcctcccaccactgccatcagggtgttaaaatttttgagctgaaggagcttctttgcaacattgataaactttgtgatgacttctgccctttgctggggggttggtttgctaagaaccatcaactggacccacttagagattccattaaataaagcaatcgatctttccaaggttggattattctccaggcagccatggatgacatagctttggtaatcagtgaatgagatccttctaaaagatttatgctccagaaaagtgaggtgctcagccaattcaatgggctccagatggtcaaacagcagacaggcttttcccttcttggatacttttttcctctgtgtgactcttctcatccagtcataggaaggaatgctggatatgtcgatgaggctgacgtgtttttcatatcctagttgactagctacttcccgaaattcctcagtcatacgaatcaaaccaagatccaaattaaactctgcaggaaacttcagaatccagtacctcatgaagtagcagatctttaatcgaaattcattgcagctttctccagtggcatttcgatacatgcagagaagtttttctgccaattcagtggaagataaataccatcggtgcatcagtagaactattcttggcaaataactattatccagctctccattgtcatcaaacatctcaatgcaagtgcacagcagttcatctaatgttgctgctttcccaaggccacttgatcccatggttatttagccgttgtcaaaaaactagagacattttcagcatcagatagaccatctccataatcatgcaagtcagcgatgttagtgcctagtggtgacctgtccttagttgtacttcaagaaaactctgttgtttccatacagatacagttccaaatctgaaagaattttaagggcagctagcatcattgggaaatgcatggaagaagcagtctgtagaactggtttattcaacctgaatgataagtattttggagaactggcccagatggtctgtatcctttctttcagaacaaaaaaaagtgggcaagcagttcctagctgcctgtgatagac

SEQ ID NO: 9034 - RNA, 1335 nt, Homo sapiens
  source 1..1335: mol_type = other RNA
actcattctcctctgtccagtctgggaaaatgacatggacagctatcaagtctttcaagtgtactccaaggatggggattttgaagccatcgcagtcggcaaaggccttgcggtaattgcagtaattgccgttggaggagaccaactctgtcatttcattccagttctttgtaacttctgaagaaagatgagaatgggtctctttgaggcgtgaaatggaactatgactgaggcctcccaccactgccatcagggtgttaaaatttttgagctgaaggagcttctttgcaacattgataaactttgtgatgacttctgccctttgctggggggttggtttgctaagaaccatcaactggacccacttagagattccattaaataaagcaatcgatctttccaaggttggattattctccaggcagccatggatgacatagctttggtaatcagtgaatgagatccttctaaaagatttatgctccagaaaagtgaggtgctcagccaattcaatgggctccagatggtcaaacagcagacaggcttttcccttcttggatacttttttcctctgtgtgactcttctcatccagtcataggaaggaatgctggatatgtcgatgaggctgacgtgtttttcatatcctagttgactagctacttcccgaaattcctcagtcatacgaatcaaaccaagatccaaattaaactctgcaggaaacttcagaatccagtacctcatgaagtagcagatctttaatcgaaattcattgcagctttctccagtggcatttcgatacatgcagagaagtttttctgccaattcagtggaagataaataccatcggtgcatcagtagaactattcttggcaaataactattatccagctctccattgtcatcaaacatctcaatgcaagtgcacagcagttcatctaatgttgctgctttcccaaggccacttgatcccatggttatttagccgttgtcaaaaaactagagacattttcagcatcagatagaccatctccataatcatgcaagtcagcgatgttagtgcctagtggtgacctgtccttagttgtacttcaagaaaactctgttgtttccatacagatacagttccaaatctgaaagaattttaagggcagctagcatcattgggaaatgcatggaagaagcagtctgtagaactggtttattcaacctgaatgataagtattttggagaactggcccagatggtctgtatcctttctttcagaacaaaaaaaagtgggcaagcagttcctagctgcctgtgatagacagctatttcacaacctccccagggtg

SEQ ID NO: 9035 - RNA, 1190 nt, Homo sapiens
  source 1..1190: mol_type = other RNA
actcattctcctctgtccagtctgggaaaatgacatggacagctatcaagtctttcaagtgtactccaaggatggggattttgaagccatcgcagtcggcaaaggccttgcggtaattgcagtaattgccgttggaggagaccaactctgtcatttcattccagttctttgtaacttctgaagaaagatgagaatgggtctctttgaggcgtgaaatggaactatgactgaggcctcccaccactgccatcagggtgttaaaatttttgagctgaaggagcttctttgcaacattgataaactttgtgatgacttctgccctttgctggggggttggtttgctaagaaccatcaactggacccacttagagattccattaaataaagcaatcgatctttccaaggttggattattctccaggcagccatggatgacatagctttggtaatcagtgaatgagatccttctaaaagatttatgctccagaaaagtgaggtgctcagccaattcaatgggctccagatggtcaaacagcagacaggcttttcccttcttggatacttttttcctctgtgtgactcttctcatccagtcataggaaggaatgctggatatgtcgatgaggctgacgtgtttttcatatcctagttgactagctacttcccgaaattcctcagtcatacgaatcaaaccaagatccaaattaaactctgcaggaaacttcagaatccagtacctcatgaagtagcagatctttaatcgaaattcattgcagctttctccagtggcatttcgatacatgcagagaagtttttctgccaattcagtggaagataaataccatcggtgcatcagtagaactattcttggcaaataactattatccagctctccattgtcatcaaacatctcaatgcaagtgcacagcagttcatctaatgttgctgctttcccaaggccacttgatcccatggttatttagccgttgtcaaaaaactagagacattttcagcatcagatagaccatctccataatcatgcaagtcagcgatgttagtgcctagtggtgacctgtccttagttgtacttcaagaaaactctgttgtttccatacagatacagttccaaattagggtggttttgtcgtggtatttttcacatcagcactctgcctgtccagctgccaagt

SEQ ID NO: 9036 - RNA, 1474 nt, Homo sapiens
  source 1..1474: mol_type = other RNA
actcattctcctctgtccagtctgggaaaatgacatggacagctatcaagtctttcaagtgtactccaaggatggggattttgaagccatcgcagtcggcaaaggccttgcggtaattgcagtaattgccgttggaggagaccaactctgtcatttcattccagttctttgtaacttctgaagaaagatgagaatgggtctctttgaggcgtgaaatggaactatgactgaggcctcccaccactgccatcagggtgttaaaatttttgagctgaaggagcttctttgcaacattgataaactttgtgatgacttctgccctttgctggggggttggtttgctaagaaccatcaactggacccacttagagattccattaaataaagcaatcgatctttccaaggttggattattctccaggcagccatggatgacatagctttggtaatcagtgaatgagatccttctaaaagatttatgctccagaaaagtgaggtgctcagccaattcaatgggctccagatggtcaaacagcagacaggcttttcccttcttggatacttttttcctctgtgtgactcttctcatccagtcataggaaggaatgctggatatgtcgatgaggctgacgtgtttttcatatcctagttgactagctacttcccgaaattcctcagtcatacgaatcaaaccaagatccaaattaaactctgcaggaaacttcagaatccagtacctcatgaagtagcagatctttaatcgaaattcattgcagctttctccagtggcatttcgatacatgcagagaagtttttctgccaattcagtggaagataaataccatcggtgcatcagtagaactattcttggcaaataactattatccagctctccattgtcatcaaacatctcaatgcaagtgcacagcagttcatctaatgttgctgctttcccaaggccacttgatcccatggttatttagccgttgtcaaaaaactagagacattttcagcatcagatagaccatctccataatcatgcaagtcagcgatgttagtgcctagtggtgacctgtccttagttgtacttcaagaaaactctgttgtttccatacagatacagttccaaattgagaatcttggcagtgaaatcagagaatccaaatgggtcatcagaggggtgccgcaggttcaggtagattgggtgtagtttccatggcaaagaagagatatggatgttttaaaagaaaatatcctttgcagaactgcaataatgttgatccctatagtgaattgtctttttctttccacttcatcacctctagcaagtttctcttcaacgtgcctaaacacctagaattcctgttctgtcttctaaaatgctgtcatcacctccattgcccaaatctagttcaaaagtgaggagagaaaaaaaattgaaatttgcaagctgtttatgcctaacaacaacatt

SEQ ID NO: 9037 - RNA, 6192 nt, Homo sapiens
  source 1..6192: mol_type = other RNA
actccaagaagaatctagacagacaggccttgctgggtgtcccactgggtctgttagcatcggatcatatcctttttgtccaatcatatttctacacagctgtccatagtttgctaaacataagcttaaagatggataatttcccctgtgtctttgggtcttcattttgaagtcttcatgtcatgtaagactatgatgaaataaatttgtatgctttttctcctattaacctgccccttgccagtgcttttcagtggaccctcagtggacacaggggaagtttccccttggccccagcagctaccagatcatggtgttctcctaacatggatagtcgactaaggtggtattcaactttgcataaaaaagattgagcgttggtcctttattcaattttcagattaaaatgcttaacacacctagagtcgactgactgaagaagagtccgggtttctctgaggaaagacttggcaataccatcacaaataatctatagtaaacattcccccaagtctttcccatgtgatccgagaacatttgccaaaatcacaagccctgggaagagagtctggccagatccttccaggactattagacatgggtcggagctgacactgataccagaactgaaacgccatcatcatcctccaagtagagtagggactaatgaagatcaatataattttccccaaatttatctgtcttcaggaaatactgcccaaggtaaaggacaagttattgcagcttgtacttcccacggctaagaaagaagcacagtgcttggtaggattcttcagggtttataggcagcatacatggcacttgaaaatacttctctggcccattattaggtgacacagaaggcactcagtcttgagtgggtcagtgagtaagacagagccctgcaacaggtccaggctacttgggccatataacccaccaaaacctagaagatcttatcatactgaaggtatctttgatggacagtaatatcatgtcgagcctcaggaaatctccgataggacactcacagcacagacccctagagtactggaatggggcctctgcctgctttttggcgaaaattaggccttcaagttagcttcaatgagcagtccctggacagactcagaacagctcaaaggccaccaaaggttagaaactggaagagccttgagaaataggccgattatgttcagagaattttgcaccattcaaaagactgcccctagcatgctattggacctgggtagagacagagcatctaatcatgggacatcaggtgactgtgtgaatggagttgcccatcattagctgggtactgtgagatccaccaagccataaggtagggtggaacagcagcccatcatccaatgagagtgctacatctaaatactggccccaagcaggtgcagaggtatgagtaagctgcacagacaagtggctctggctcccaggtcattgtccctgatgcaccaatgcttcctccttagcttatacctatggacttgaatagcatgtcctatgaccagctggcagaagaggggaaaaaattaggcctggttcaaaaacagattggcgttacatgtcagtgagagcctaaaatggatgattgctttaccgcagccacactgagggatgatatcaaaagcctgcagtgagaggagattctcccaatggccagtgccatgggtcagccactctgggtggaaaaagagacagcctgggataaggatatgcctgaactcctgggaaataggaaatggtttggttggttggtcagcgacctggaagaagcaatattggaagatttgcacaaggggatctgggtaaggagctgtagatggacctctgggactgggcacaaggtgtaaggatcttggtgtttcatgttagtgtccactgaaaagcatccaatatataagaggcactaggcaaccaaatggactggcacattcagcccatgggtatcagacaagtttgatcttcaactaccctagtgcttatacaatgggcccataaatggagtcgctatggtggcaaggatggaggctatggagggcccaacatcatgcatgggctctccccaactcacaaagctgatctaatgactgccactgaatgtccagtctgtcaacatcagtgtccagaagagtcctccagatgataccatccctgaagagaccaaccaaccacttggtggcaaatggattacataagacaccttctacctgggaaagggcggtgattcattctgttctaaattggcatgcattccaggtgtgaattcacctttcctgccctcagtgcctcagtagcaccactaaccagagacctacagagtgtctgatttaccaacttgagatcccatataacatcgtcttaggccaagaaatccactttatggcaaagaaggtataggaaagggcataaaaccacaatattcactgatcctgacacatcctgctttctccagaaggtgccagcctgagagggccttggatcaggctcttgcaggagctgctgaggcactaacattgtgaagctggtgtgtggtctttcaggatgtggtatatattttaagccaatggccattgtctgatgctgttactattttccaataagtaaagggacaggcattatcagatttacactttagatagattatttcagcagtagtgtggaatatagatttgaaagtgggaaaagaatggaggctcctttagcaaccaagaaccaaggggcggagggagaagtggtcccactcattatcatccccagtagtccatttggggagttgtgcttctcatccctgtaacttaggttctatgattctagagatcatgagtcccagagcaggaacatagtaagagtcccactaaacctaaagatatggcgtccaccttagattgcacctatggacttgacagcatgtcctatgataagctgacagaagagcatctttgtacagaagatcagcaggtaaataaaagagttaccatctcctggtaatcattggcccacgttgttatgaagagatgggactggagccacactaagaaggaactcacgggatccactggtgttactgttgcttgctacacagaaagctaatcactgagacaagccagggaagaaggctttattattttataggtgacatcagctggagagatgggagccaaacctcaaatctatcctgccgtgccccctcccctcaactaaagtgagggatttaaatatcaggagggacaaggaagaagagttggtcaaccagcagccaattcctttcattgtacaaatgtaagtttctcaagcttcagttctgtgggcatctggcttgttggaaaactgggctgatttcacagggacgtgtctaggcgttctctcacctagttttgactgggaatgggcaagtgcaacaccacagcctgatgagagcacggcaagtaggggtgcagacccctcgggggtaaaggtctgtcaggccaccaggcaacccacggagagcagcagaagtgcaggagaaggaggcagggaatctacagcgacggcagaggcggggcacaataaatatcagttacggtgtcaggagtcatttcagcagcagaggctataacttgtcccactaatcttcctcctttaagtatttccttaggatttgtgacaagccaccatcttgaaggagccccgaccaggaggagtgagcttggtgtgagatgcaagcatagctgagcagttgcagggggtggattgtagctgaccccactggtcctctgctcaggtcccctaggacccctctgactgtttgtgagcccattacacagcttttgcatgctcttgcctgcagtggcccatacatgctacttgtgagctattggagagtttacctgcatcccacccacacctgccacgaggcgacccttagccgatgcctgatgggtgccaaagtgtaaaaacccagctctcttgcttgaacggaaacaaaactgagatgtggtttgcactccaaaattgctctgtgggctcgctgcagctggaactttggatgcaaatccttgcttggcttcctccttcccttcccacttccaacatcccttgctggttcctcttgggacctgtgccctcatcaatcacacacccctgagtcctcctctcagaggctgcttctgatctcaaacagcctctgctgtgtgctgggccatgctcctaaacgtggctttccccagccgcaccagcaccagctcctgaggcactccatcagcccggcatcgttgcacactcctggcccgaacccccttattctcatgccccaatcgtaggccccctcggggttcttgctcaagctgacaccccgccgggaaggcttgctctcttctctcctcaactcagtcctcatcatcctgctctctaaagcctcctcccacgcttctgatcccaagtggcttccacgcctctgaattcctgtcacattcatatccaagaccacccccaaacagtgtaacgtcagcatctgtggcagaggggagagaagccccaggaggtgtcgtctgcctgccttttggtgcaagctggtgtatgagtcgatcaggctgaaccgagcaccactgaccgggcagcttaagcacagcttatttcctcgcgactctggaggcgggaagtctgagacgcaggtgccggcaggctcagttcctgcagagacctgtccgcggcttgcagacggccatcttccgtgtcctcacagggtcttccccatgtgtgtctgtgtcctcatttcctagtcagattggatgagggcccactttaattacctgtttgaagacactatctccaaatacattctgaggtgccgggggttaggacatgtaaattctgggggatacaactgagcccgcacatcaggctctggcttgagcctcagggagcatccctgtgtgactccgaactgctcaagagcgtgggggtcaggaactgggggagcgcttaggagtggacctgatcactcgctcagcggtccctctcccccgcttgcccaccttccttcccataggtgctgacttcagacagacaggacttgactcctggctctgtctcccggatcggacgcgtgagaggctacttaatctccctgggcctcgattccctcgtccatgaaatgagggtgatgccctctatcttagtgagccccagagaaagacactggtgtgaagacgccggcctggggcaagtgtgcaccagggccccgctgtttcttcccccagggcgacttccaagcctgcgaatgccggctcttgtttggggactcccacaaacgtttacacgggatttggataacctacaattcttgacttaagcttcattaggattttaaactccgaggggagagctcatgtctgactttcttcgtattccaccgaacagggccagggcagagaggcctctctgcttgtggactctggtccctgcacttcagtcctgttgtcaccagacattatctcagcaaccacagacacctcagggaaatccgcccttcaccgcgagccaggagtgtcctgccccagactttcccacagggccatgaccaccctggaagcacagcgctgctcagtgggctgcggtcctgggcccttatctcatcagcacacaagcccgttattcagccgtatttacataacccttccctcccgcctgcctcccacctccagctgctccctgggcacaaagctccggtttcacttaatcaaccatgcagtctggtgtcccaggtaacaagccatccatttgtgttggcagcatttgaaggtgaggggcagataaccctgagccctgccagtggctccgctgacagcactgggagtcctgggccacttcctcaagcaatacatccagagcaagggttcctctgggaacacaaaatcactccctctgtgtccagactcacatgataagacttcttacagcagctcactttcctctgaggacagaacgcaggacaaccagggcacctgtctgtcttgatggcatcttcccccacacgctttccatggagcagcagcagatgacaaccttcaccatgcacaaacgccatgcccagcccttcacacgcggtgcacagtggctcacacactgtggtgcatcaaggagcatctcacacggggtgttgcacagagtaccacggagtatcacacacag

SEQ ID NO: 9038 - RNA, 220 nt, Homo sapiens
  source 1..220: mol_type = other RNA
actccaagaagaatctagacagacaggccttgctgggtttcctcactccatctgttaaagttacatcatacccttttgtccagtcatatttctaaacagctctacatactttttgaacctaagcataaaaatgtgcactttcctctgtcttcattctgaaggttcccatgtacacattaaatgcatttgtatgttatttctcctactagtctgccttttg

SEQ ID NO: 9039 - RNA, 1108 nt, Homo sapiens
  source 1..1108: mol_type = other RNA
actccagccccacagcctcagcctggccctggcattgccctggcatttgctcactgcgtggtggttggacggtggcaggcccttctccacactggggggcacgtcatacacctccagcaacgggtctcggccattgggacccttgacagccatggggggtgtgtcatacacctcctggccatactggctgggaagcagcccccgaaccgggggcacatcatagatgtcctgtggccccggggccagcaggtgtcgcgggatgtcgtactcgtcctgctccggctgggcggcctcgtatacatagccctgccccacgcgggtgggcaccaccacctttgccgggggcttcgtgccctcccagctgcgtgtgtccatggacggggggacctggtagatgtcatgccccatcccggcagaaggtggcacctggtaaatatcctgggcagggcctccaggccctgggggcacctggtacaggtctgtggccgggctgggaaacgggtgatggggtgtctgcttcgagaaggtggatgtctgcttggctgggggagactggaactgagggctgggacccgggacttggtagaggccttgctgagccttgctgggagtgggcaccaggtagacgctgtctggctggggctggtaggtgttggggagcatgggcgtgtactgggaggccggaggcgctggggcatggaggccaggctgaggctgggccggggtggcgggagggccggggccaggccctgctggcttcttatcatacatgcccaccaagatcttgaggcggttcccaggcacgatgccctggcgcccatgcagcgagcagagccaccagccgtccaggccctgcgtgtcctgctccagcaccgtcatgatgtcacccttgcggaaggagagctcatccggggactcggccacattgtcatagagcgctttggccagcacgttcaggtggttcatggtgtccggcgggcctggggccccggctctcgcgggggcgcacaccgagctgcccgggccgcgtgccctcggggctccgagcgcgccgcagccgccccggtgccgccgcgcagctgccgcctcggccacccagagccggtcc

SEQ ID NO: 9040 - RNA, 2181 nt, Homo sapiens
  source 1..2181: mol_type = other RNA
actccatttgttttgatgatggacctttgatctttgggttttggtggcacaggacctacaaatccaatattgtcataaaagttatgaatagcgctggggttaaaatgtggtcctcgggcttgaaaaagatcaatttctttggttaagcagtcaatgtcaatctggagttgtctattacaacttctcagctgctgcatttcttcaagggaaggtatctgggatatagaatttgatcttttcaggcgccttcgagttagattattttccatttcattaacctcagattttaatttatccagctttttcttttgaatctcaagttctctttgaagtcgttccattctggccttctggtgtaccaaaagagcttgtgtgtaggcagcatcatcagatcccatactcagtttccgtgtttcacttattctatccacatgtgctaatgtagggtccgtgaggtgctgaatattctcggtttctacataatgatcaggatgattaagaagatttgtaagttcaaaggtaggggacaccacccctggtgaaactgcagggggcttattgggagagactgtaattttgaaagtgtatttcgtattgggctgagtgactaccactcgaggagaggttgcagagttattgcctattgctcgacttttgggaggatggtgatgaataaaggcaggacccatgctcacttgcccagacatgttcctggaggcagcagatgctccagagtttgtggatatgaagagtgtgggctgattccgcatgacctgttcatctcctgtggcagcattcgctgaaatatagaccttaggttgactacgggacatcagctcatccgtatttggggggctggcagctatgtaaacagtgggctgatttctgtttaaggtctggctattgactgaagaggaagtgctggaggttcgaggtccagaagaacgcagttttgaagaattatttctttgtgggggttcaagtttgatttcaatctggttttttcgaggtcctgttgaaatattctgaatgttatattggctatgggcagaagactgtgagctaccagatgaatgaatggttggtggttgtgaagtagtaggtgaactgattggcatgtagacatgagaggtctggtggccttgctgatttggctgttgagatgaggtatgtgacagaggattagatgcaggacaagtagtccagggaccaggctgtgaaggctgataaacttgctgagggttcatgggattaaactgagatacccagccagaatgctgttgtgtctgtcgagttgtaccaccaggagttgtaatgtaaggcctaatatagatagaatttccctgtggactgttaagtacaggtggaggtacaccatgtatgtgcaaagatgtaggagtattacgaccagtctggatatttggggctaaagttaccataatgggattaaatctgggagtttgttgagaaaggctagatgttcctttgctgcctaagtgaaatccaagatgtggtgctgaatttgaagcaccagaggaactggacattccaaaaacattaaagccttgaggaacttgagctggtgctgtctgtggctcctgctgaaatagttcactattggactggccaccttgaagttgtccatcactaatgctgtgcgttagagtcctacttccattcatcctacttccttctcttccatggtggtaaatgttctgtgattgcaagtccaagttgagagaagtcatgtgattgcgtagaccagaaattccagaatcatctgaaaaattcaagtctccttcaccataaagatatcttgtactctcctgagagagaacagcacagcaggcatccaggttattattattctgcattctcagttggtttgctttggaggaataaacttagtctcaaatccttcttcatccaggcagtcatattgaaactggatcagatggtgtttagatctttacagcctgtggccctgaaggagttcacctcactgagcattagtcttctcatcaggttagtatgcagttctgcagctcagggacctaggctcctcttgtctcgtagttctgctatgaatggcctccattctcatggttgttgtcatattctgagactgttgctccagcttcagcttttgcctccatacttaacatttcagactccagaaag

SEQ ID NO: 9041 - RNA, 2898 nt, Homo sapiens
  source 1..2898: mol_type = other RNA
actccatttgttttgatgatggacctttgatctttgggttttggtggcacaggacctacaaatccaatattgtcataaaagttatgaatagcgctggggttaaaatgtggtcctcgggcttgaaaaagatcaatttctttggttaagcagtcaatgtcaatctggagttgtctattacaacttctcagctgctgcatttcttcaagggaaggtatctgggatatagaatttgatcttttcaggcgccttcgagttagattattttccatttcattaacctcagattttaatttatccagctttttcttttgaatctcaagttctctttgaagtcgttccattctggccttctggtgtaccaaaagagcttgtgtgtaggcagcatcatcagatcccatactcagtttccgtgtttcacttattctatccacatgtgctaatgtagggtccgtgaggtgctgaatattctcggtttctacataatgatcaggatgattaagaagatttgtaagttcaaaggtaggggacaccacccctggtgaaactgcagggggcttattgggagagactgtaattttgaaagtgtatttcgtattgggctgagtgactaccactcgaggagaggttgcagagttattgcctattgctcgacttttgggaggatggtgatgaataaaggcaggacccatgctcacttgcccagacatgttcctggaggcagcagatgctccagagtttgtggatatgaagagtgtgggctgattccgcatgacctgttcatctcctgtggcagcattcgctgaaatatagaccttaggttgactacgggacatcagctcatccgtatttggggggctggcagctatgtaaacagtgggctgatttctgtttaaggtctggctattgactgaagaggaagtgctggaggttcgaggtccagaagaacgcagttttgaagaattatttctttgtgggggttcaagtttgatttcaatctggttttttcgaggtcctgttgaaatattctgaatgttatattggctatgggcagaagactgtgagctaccagatgaatgaatggttggtggttgtgaagtagtaggtgaactgattggcatgtagacatgagaggtctggtggccttgctgatttggctgttgagatgaggtatgtgacagaggattagatgcaggacaagtagtccagggaccaggctgtgaaggctgataaacttgctgagggttcatgggattaaactgagatacccagccagaatgctgttgtgtctgtcgagttgtaccaccaggagttgtaatgtaaggcctaatatagatagaatttccctgtggactgttaagtacaggtggaggtacaccatgtatgtgcaaagatgtaggagtattacgaccagtctggatatttggggctaaagttaccataatgggattaaatctgggagtttgttgagaaaggctagatgttcctttgctgcctaagtgaaatccaagatgtggtgctgaatttgaagcaccagaggaactggacattccaaaaacattaaagccttgaggaacttgagctggtgctgtctgtggctcctgctgaaatagttcactattggactggccaccttgaagttgtccatcactaatgctgtgcgttagagtcctacttccattcatcctacttccttctcttccatggtggtaaatgttctgtgattgcaagtccaagttgagagaagtcatgtgattgcgtagaccagaaattccagaatcatctgaaaaattcaagtctccttcaccataaagatatcttgtactctcctgagagagaacagcacagcaggcatccaggttattattattctgtaacatgcacctggatacaacaacttcaggtacttcagggaatttttgtcgcaggtcatgtaaaacctgaaaatcaatttggtggcttccttgggccattcgtatattgcctgatcaggactatttgtacagtaggcaattctaggccttagtggaaatagtactcatctcttctgtccaagcattttcagttataagttcttctaaaaggaatgtgcaagtcggccacacttggcaatttatgtactgtggttttgtggtaggtactacattttctggaaatagaaaaattcaaattgtagctgttcttggttggcccattgccatttttgcagcttacaaattgttaattaagtaactgcagtgagctcatctctacgggatacttcttttccagggcaggtccaggaactgggtctggagccttgaaagcagaagagaaactagagtaaactagaggtaggcagaacaagaaatgtgaccagataacattatgagatgtaatagcagtaaggtagtccccaaagtctctcacataaaatattctgaagggaaaatgggtctcttaaattgcaagtaaccaaaggatgctgtttactttggttaagccattcttttaacctacccaacactattctggaatctcagttccagcaactcaaaacagtagtttttatgaaatctctaatggcttttagcaacagactgtccaacaggagaccacagagtaactctaacagaaagagaaaaacaacaacaaaatccaaaattggaaatgtaaagtcctcattttcaggtcatttttctcttccctttcactatcgtatttccaatcatcttctaaacgctcccctaatttcctatgatccattcccaggggtttcttaagaaatgctttagatatatccaagcaatgaattgaatgttaagttccaatttttaaaaatacttggtaattcttaaagagggaggcaaagaacagctcataagatgtggttcttaaccacactggaaaatctttttttcc

SEQ ID NO: 9042 - RNA, 2363 nt, Homo sapiens
  source 1..2363: mol_type = other RNA
actccatttgttttgatgatggacctttgatctttgggttttggtggcacaggacctacaaatccaatattgtcataaaagttatgaatagcgctggggttaaaatgtggtcctcgggcttgaaaaagatcaatttctttggttaagcagtcaatgtcaatctggagttgtctattacaacttctcagctgctgcatttcttcaagggaaggtatctgggatatagaatttgatcttttcaggcgccttcgagttagattattttccatttcattaacctcagattttaatttatccagctttttcttttgaatctcaagttctctttgaagtcgttccattctggccttctggtgtaccaaaagagcttgtgtgtaggcagcatcatcagatcccatactcagtttccgtgtttcacttattctatccacatgtgctaatgtagggtccgtgaggtgctgaatattctcggtttctacataatgatcaggatgattaagaagatttgtaagttcaaaggtaggggacaccacccctggtgaaactgcagggggcttattgggagagactgtaattttgaaagtgtatttcgtattgggctgagtgactaccactcgaggagaggttgcagagttattgcctattgctcgacttttgggaggatggtgatgaataaaggcaggacccatgctcacttgcccagacatgttcctggaggcagcagatgctccagagtttgtggatatgaagagtgtgggctgattccgcatgacctgttcatctcctgtggcagcattcgctgaaatatagaccttaggttgactacgggacatcagctcatccgtatttggggggctggcagctatgtaaacagtgggctgatttctgtttaaggtctggctattgactgaagaggaagtgctggaggttcgaggtccagaagaacgcagttttgaagaattatttctttgtgggggttcaagtttgatttcaatctggttttttcgaggtcctgttgaaatattctgaatgttatattggctatgggcagaagactgtgagctaccagatgaatgaatggttggtggttgtgaagtagtaggtgaactgattggcatgtagacatgagaggtctggtggccttgctgatttggctgttgagatgaggtatgtgacagaggattagatgcaggacaagtagtccagggaccaggctgtgaaggctgataaacttgctgagggttcatgggattaaactgagatacccagccagaatgctgttgtgtctgtcgagttgtaccaccaggagttgtaatgtaaggcctaatatagatagaatttccctgtggactgttaagtacaggtggaggtacaccatgtatgtgcaaagatgtaggagtattacgaccagtctggatatttggggctaaagttaccataatgggattaaatctgggagtttgttgagaaaggctagatgttcctttgctgcctaagtgaaatccaagatgtggtgctgaatttgaagcaccagaggaactggacattccaaaaacattaaagccttgaggaacttgagctggtgctgtctgtggctcctgctgaaatagttcactattggactggccaccttgaagttgtccatcactaatgctgtgcgttagagtcctacttccattcatcctacttccttctcttccatggtggtaaatgttctgtgattgcaagtccaagttgagagaagtcatgtgattgcgtagaccagaaattccagaatcatctgaaaaattcaagtctccttcaccataaagatatcttgtactctcctgagagagaacagcacagcaggcatccaggttattattattctgtaacatgcacctggatacaacaacttcaggtacttcagggaatttttgtcgcaggtcatgtaaaacctgaaaatcaatttggtggcttccttgggccattcgtatattgcctgatcaggactatttgtacagtaggcaattctaggccttagtggaaatagtactcatctcttctgtccaagcattttcctttgccgccgccgcttccccctcctcctcctcggccgccgccgccgccgcctctcccactagggcagccgtctccaccgtcgcctccgccaccacggccgccgccagcgccgccgccgcctccggttccacccggcaggggggacacctcagccctccctccctccccgctcagccccctccgctcgcccgccgccgccaactccctccggccgccgccgccgccaccgctcctggctgagggggaggggagggggtcgggctgggtcgccccgccggcggctgcagcagatcaaaaacgac

SEQ ID NO: 9043 - RNA, 2512 nt, Homo sapiens
  source 1..2512: mol_type = other RNA
actccatttgttttgatgatggacctttgatctttgggttttggtggcacaggacctacaaatccaatattgtcataaaagttatgaatagcgctggggttaaaatgtggtcctcgggcttgaaaaagatcaatttctttggttaagcagtcaatgtcaatctggagttgtctattacaacttctcagctgctgcatttcttcaagggaaggtatctgggatatagaatttgatcttttcaggcgccttcgagttagattattttccatttcattaacctcagattttaatttatccagctttttcttttgaatctcaagttctctttgaagtcgttccattctggccttctggtgtaccaaaagagcttgtgtgtaggcagcatcatcagatcccatactcagtttccgtgtttcacttattctatccacatgtgctaatgtagggtccgtgaggtgctgaatattctcggtttctacataatgatcaggatgattaagaagatttgtaagttcaaaggtaggggacaccacccctggtgaaactgcagggggcttattgggagagactgtaattttgaaagtgtatttcgtattgggctgagtgactaccactcgaggagaggttgcagagttattgcctattgctcgacttttgggaggatggtgatgaataaaggcaggacccatgctcacttgcccagacatgttcctggaggcagcagatgctccagagtttgtggatatgaagagtgtgggctgattccgcatgacctgttcatctcctgtggcagcattcgctgaaatatagaccttaggttgactacgggacatcagctcatccgtatttggggggctggcagctatgtaaacagtgggctgatttctgtttaaggtctggctattgactgaagaggaagtgctggaggttcgaggtccagaagaacgcagttttgaagaattatttctttgtgggggttcaagtttgatttcaatctggttttttcgaggtcctgttgaaatattctgaatgttatattggctatgggcagaagactgtgagctaccagatgaatgaatggttggtggttgtgaagtagtaggtgaactgattggcatgtagacatgagaggtctggtggccttgctgatttggctgttgagatgaggtatgtgacagaggattagatgcaggacaagtagtccagggaccaggctgtgaaggctgataaacttgctgagggttcatgggattaaactgagatacccagccagaatgctgttgtgtctgtcgagttgtaccaccaggagttgtaatgtaaggcctaatatagatagaatttccctgtggactgttaagtacaggtggaggtacaccatgtatgtgcaaagatgtaggagtattacgaccagtctggatatttggggctaaagttaccataatgggattaaatctgggagtttgttgagaaaggctagatgttcctttgctgcctaagtgaaatccaagatgtggtgctgaatttgaagcaccagaggaactggacattccaaaaacattaaagccttgaggaacttgagctggtgctgtctgtggctcctgctgaaatagttcactattggactggccaccttgaagttgtccatcactaatgctgtgcgttagagtcctacttccattcatcctacttccttctcttccatggtggtaaatgttctgtgattgcaagtccaagttgagagaagtcatgtgattgcgtagaccagaaattccagaatcatctgaaaaattcaagtctccttcaccataaagatatcttgtactctcctgagagagaacagcacagcaggcatccaggttattattattctgtaacatgcacctggatacaacaacttcaggtacttcagggaatttttgtcgcaggtcatgtaaaacctgaaaatcaatttggtggcttccttgggccattcgtatattgcctgatcaggactatttgtacagtaggcaattctaggccttagtggaaatagtactcatctcttctgtccaagcattttctggaaatagaaaaattcaaattgtagctgttcttggttggcccattgccatttttgcagcttacaaattgttaattaagtaactgcagtgagctcatctctacgggatacttcttttccagggcaggtccaggaactgggtctggagccctttgccgccgccgcttccccctcctcctcctcggccgccgccgccgccgcctctcccactagggcagccgtctccaccgtcgcctccgccaccacggccgccgccagcgccgccgccgcctccggttccacccggcaggggggacacctcagccctccctccctccccgctcagccccctccgctcgcccgccgccgccaactccctccggccgccgccgccgccaccgctcctggctgagggggaggggagggggtcgggctgggtcgccccgccggcggctgcagcagatcaaaaacgac

SEQ ID NO: 9044 - RNA, 2391 nt, Homo sapiens
  source 1..2391: mol_type = other RNA
actccatttgttttgatgatggacctttgatctttgggttttggtggcacaggacctacaaatccaatattgtcataaaagttatgaatagcgctggggttaaaatgtggtcctcgggcttgaaaaagatcaatttctttggttaagcagtcaatgtcaatctggagttgtctattacaacttctcagctgctgcatttcttcaagggaaggtatctgggatatagaatttgatcttttcaggcgccttcgagttagattattttccatttcattaacctcagattttaatttatccagctttttcttttgaatctcaagttctctttgaagtcgttccattctggccttctggtgtaccaaaagagcttgtgtgtaggcagcatcatcagatcccatactcagtttccgtgtttcacttattctatccacatgtgctaatgtagggtccgtgaggtgctgaatattctcggtttctacataatgatcaggatgattaagaagatttgtaagttcaaaggtaggggacaccacccctggtgaaactgcagggggcttattgggagagactgtaattttgaaagtgtatttcgtattgggctgagtgactaccactcgaggagaggttgcagagttattgcctattgctcgacttttgggaggatggtgatgaataaaggcaggacccatgctcacttgcccagacatgttcctggaggcagcagatgctccagagtttgtggatatgaagagtgtgggctgattccgcatgacctgttcatctcctgtggcagcattcgctgaaatatagaccttaggttgactacgggacatcagctcatccgtatttggggggctggcagctatgtaaacagtgggctgatttctgtttaaggtctggctattgactgaagaggaagtgctggaggttcgaggtccagaagaacgcagttttgaagaattatttctttgtgggggttcaagtttgatttcaatctggttttttcgaggtcctgttgaaatattctgaatgttatattggctatgggcagaagactgtgagctaccagatgaatgaatggttggtggttgtgaagtagtaggtgaactgattggcatgtagacatgagaggtctggtggccttgctgatttggctgttgagatgaggtatgtgacagaggattagatgcaggacaagtagtccagggaccaggctgtgaaggctgataaacttgctgagggttcatgggattaaactgagatacccagccagaatgctgttgtgtctgtcgagttgtaccaccaggagttgtaatgtaaggcctaatatagatagaatttccctgtggactgttaagtacaggtggaggtacaccatgtatgtgcaaagatgtaggagtattacgaccagtctggatatttggggctaaagttaccataatgggattaaatctgggagtttgttgagaaaggctagatgttcctttgctgcctaagtgaaatccaagatgtggtgctgaatttgaagcaccagaggaactggacattccaaaaacattaaagccttgaggaacttgagctggtgctgtctgtggctcctgctgaaatagttcactattggactggccaccttgaagttgtccatcactaatgctgtgcgttagagtcctacttccattcatcctacttccttctcttccatggtggtaaatgttctgtgattgcaagtccaagttgagagaagtcatgtgattgcgtagaccagaaattccagaatcatctgaaaaattcaagtctccttcaccataaagatatcttgtactctcctgagagagaacagcacagcaggcatccaggttattattattctgtaacatgcacctggatacaacaacttcaggtacttcagggaatttttgtcgcaggtcatgtaaaacctgaaaatcaatttggtggcttccttgggccattcgtatattgcctgatcaggactatttgtacagtaggcaattctaggccttagtggaaatagtactcatctcttctgtccaagcattttctggaaatagaaaaattcaaattgtagctgttcttggttggcccattgccatttttgcagcttacaaattgttaattaagtaactgcagtgagctcatctctacgggatacttcttttccagggcaggtccaggaactgggtctggagcctgtaatcgcagcactttgggagaccaaagcaagaggatcacttgagccaaggagtttgagactagcctgtgcaatacagcaaaaccctgcctctgggggcgggtcaggggcgccgacgcagggaggggccctcccgagccccttgcgccctcccccacccggggctctcctaggcgctcgat

SEQ ID NO: 9045 - RNA, 2830 nt, Homo sapiens
  source 1..2830: mol_type = other RNA
actccatttgttttgatgatggacctttgatctttgggttttggtggcacaggacctacaaatccaatattgtcataaaagttatgaatagcgctggggttaaaatgtggtcctcgggcttgaaaaagatcaatttctttggttaagcagtcaatgtcaatctggagttgtctattacaacttctcagctgctgcatttcttcaagggaaggtatctgggatatagaatttgatcttttcaggcgccttcgagttagattattttccatttcattaacctcagattttaatttatccagctttttcttttgaatctcaagttctctttgaagtcgttccattctggccttctggtgtaccaaaagagcttgtgtgtaggcagcatcatcagatcccatactcagtttccgtgtttcacttattctatccacatgtgctaatgtagggtccgtgaggtgctgaatattctcggtttctacataatgatcaggatgattaagaagatttgtaagttcaaaggtaggggacaccacccctggtgaaactgcagggggcttattgggagagactgtaattttgaaagtgtatttcgtattgggctgagtgactaccactcgaggagaggttgcagagttattgcctattgctcgacttttgggaggatggtgatgaataaaggcaggacccatgctcacttgcccagacatgttcctggaggcagcagatgctccagagtttgtggatatgaagagtgtgggctgattccgcatgacctgttcatctcctgtggcagcattcgctgaaatatagaccttaggttgactacgggacatcagctcatccgtatttggggggctggcagctatgtaaacagtgggctgatttctgtttaaggtctggctattgactgaagaggaagtgctggaggttcgaggtccagaagaacgcagttttgaagaattatttctttgtgggggttcaagtttgatttcaatctggttttttcgaggtcctgttgaaatattctgaatgttatattggctatgggcagaagactgtgagctaccagatgaatgaatggttggtggttgtgaagtagtaggtgaactgattggcatgtagacatgagaggtctggtggccttgctgatttggctgttgagatgaggtatgtgacagaggattagatgcaggacaagtagtccagggaccaggctgtgaaggctgataaacttgctgagggttcatgggattaaactgagatacccagccagaatgctgttgtgtctgtcgagttgtaccaccaggagttgtaatgtaaggcctaatatagatagaatttccctgtggactgttaagtacaggtggaggtacaccatgtatgtgcaaagatgtaggagtattacgaccagtctggatatttggggctaaagttaccataatgggattaaatctgggagtttgttgagaaaggctagatgttcctttgctgcctaagtgaaatccaagatgtggtgctgaatttgaagcaccagaggaactggacattccaaaaacattaaagccttgaggaacttgagctggtgctgtctgtggctcctgctgaaatagttcactattggactggccaccttgaagttgtccatcactaatgctgtgcgttagagtcctacttccattcatcctacttccttctcttccatggtggtaaatgttctgtgattgcaagtccaagttgagagaagtcatgtgattgcgtagaccagaaattccagaatcatctgaaaaattcaagtctccttcaccataaagatatcttgtactctcctgagagagaacagcacagcaggcatccaggttattattattctgtaacatgcacctggatacaacaacttcaggtacttcagggaatttttgtcgcaggtcatgtaaaacctgaaaatcaatttggtggcttccttgggccattcgtatattgcctgatcaggactatttgtacagtaggcaattctaggccttagtggaaatagtactcatctcttctgtccaagcattttctggaaatagaaaaattcaaattgtagctgttcttggttggcccattgccatttttgcagcttacaaattgttaattaagtaactgcagtgagctcatctctacgggatacttcttttccagggcaggtccaggaactgggtctggagctcaggttttttagctttctgagtaagcagcgtccttgattttttaggaccagaatcataagaaacaaaatgttaaaatactgttaagtattctggaaatatgagccagaggcaaaaacatatgaacatgcatacatttaaattctatataatttcaatgtctccaaatccttatcattttaatacagagggttttaaataagatgacatatatagagtgtcagaacctatgaaaaggttcagagacaatctcctttgtacagttcagcatgatcattttcctgtgcttggcagccaccactacccacatctccacattcctagctgcctaaaacttttcatctaattctctgctagcatcttatcctctgtctctcctcctccttattactgttttgcccaatcttcacatgtgcctctgttattacctcataatccttccattctagagagacccaatgttagatcaaataaagatgacataagtgaaacaaaggaaaagtgctactagtgttctctgggtcatgggaacctggccagagagagatataatggaattataatttggatttttcaattacagtttaatttatgaactttatatattataaagattatcagga

SEQ ID NO: 9046 - RNA, 435 nt, Homo sapiens
  source 1..435: mol_type = other RNA
actccatttgttttgatgatggattcttatgctccatcatcgtctcaaatgagtcttcagagggttctatcatttcgtcggatggaaaggagtgtattctgaagattggtaaggttgtgatggcgtccagtcagtagctgggaccgtggagatcagaaccttggctgcaagcgttcaagtggatctcctcccgtcctgtgccactcgatcctcgctgcttgcttccccgggcccagtcccaagcgtgaggctggggatgaagtgatgccggtggcttagtgatgccggtggcttcctgtcctcgaagctcagtcggtcgtctctcagctggtgtgaggctgggccaggatggaaccccagactctccgaggctccccaccacaccctgctgctgaaggctgctcagcgaggctgtgccgagtgctgggggggtgt

SEQ ID NO: 9047 - RNA, 138 nt, Homo sapiens
  source 1..138: mol_type = other RNA
actgacaggagagcattttgaaacgcaaggtcagaaaggttaaaggaagcaagtatatgaaaagtgattttttgttgttgagactgggtctcacccagtcacgcaggatggagtgcagtgacaggacctccagagctc

SEQ ID NO: 9048 - RNA, 349 nt, Homo sapiens
  source 1..349: mol_type = other RNA
actgacaggagagcattttgaacttgcacacagcaatcaggatgaatgtcaccccaactgacagcaggacgggcccaaggagctgggtccattcaaagtgggagacaccttggtatttgatccagcccatgacagtgaatgtgatccccaccagtcccagaaagatgcctgagaagagcaaggtggcccccgccttgtcatcatcggacacctggatgtcagcggtgctgggtgtgtaaggagtgacggagaacacattgacagggaagtcctccaagcggccgctgccctgctccattgctccttgtgggctcaccctgcttcttagagtggagaggattgtgagaac

SEQ ID NO: 9049 - RNA, 8789 nt, Homo sapiens
  source 1..8789: mol_type = other RNA
actgagcctctctctctccagagagcatctcagctctcgtttttgggtgtgcagggcttccaccgtcgacttcagtgtggcacttacctccttctctctcctgagcgcctcacagtgcttctgagcctcagcctcaagctgctgctgagaatgcagggcttgctgctgcaccttttcaagcatcgcttgcaagtccaccacccgggacttctcctccttcagcttctgcagcagagcgtgatgggcctgtgtgtcctggtgcacgcaagcctcctgtgtcctctggctcagctgctcggtcaggagccgctcgtgccgcaaggcctctgacagctccagggtgcggctcttctcagccgcaaggtccttctggagctcagagagctggctccgctcctgagccagcaaggcctcgcagcgtgagtgctcgatacgcagctccttctgcaggttgtccttggccgtctgctcgtgtttcagtgccacgcagagtcgactgctctgagcacgctgtgtctccaaagacgcccgcagctcctccagggccttggcactctggctctccctctgcaggtgccgcagctgctcctcctccagctggctctgcagggcacgccccttcccctgctcactctccagctcctgaagcgcggccttcagctcgttctccttactgctcagcatggatctcagctggaggacctcctgctgcacctcgcagagggaccgggacagctgttcgctcttctgcctgctctcacagaggtcggacttcaaatctcgcactacagtctgctccgccgccaggagcttctgcacgctgtttgccttctcttgctcttcactcagcgtcttctgcaagtcaccagcaatgcacttctcctgctctactttataagccagcagttcaacctgcctgcgcagctggtgctcctgctggctcccgcgcgcctctgcgcttgtcagcgccgtgcgcaagtgctgcagcttctcctggttctgcaggtgcgtcatgcgcagctgggcacgcagcgcctggatctcggacagcaggctgctccggtccggcaagcgaagatgctccagggacttttcctgcaggtctccctgctcacggatgatcttctccagcctttcgagcagggagctgtgaccccccagatctgagccactgagtcggggctgcagctcaaccccctgcatctcctgctctttttcaaaggcctcttgcacaacctgcagaaggtcccctctccaatcggggcacgcggtgggcacttcctgcgtctttcccccatggagcgagatgtcctgtatctcgtcttccttccggggtgggtgtggctcgccgcttgggggtgcaaggccttctgacagcgccaggatctggtggctctcgtcacgcaccatctgcagtaaagccttcacgtgcttcggacgcacttccttctccttcatggcttccggcagcggctgaaaccttccagagatggaagcaggggtcacaggaccagcagtttgagcctcagggcctcctgaccccgggctcagtcttgctccaaaacccgagccgtcacttttctcacttctatcagcttttccttctaatccaggaggaggtgaacttaatgtttcttgagaatcaaaggatgttgtgataaaatcttcgacatctttctccacagccgtcctctgcacatggtggtcgtcagccggcggagactcggcccactgcagtgccagcgctgctgcagacacgcctggggaacaaagcagccccggcccctgggtctgtggcagcgaggtgtccgccctgtcccccagggatgtgtcggcactgcacaggctcagggctcctgagtggggtgtcacggggaggctgggccagggctccagggtccagtccttcctgaggacctcaggggagctccaggaagacaggtccagcatcccgaccgggctcttccggggcccagcctctgcagtgtggctctggtggcgggagccaccaagtacgctggtcggtgaagaaagagacatgtcctgacattctgatttttcttgaatgggagaatctggcatttcatctggtatcaaggaatcccaatttttgataacatcagttacaccccctggggttgtattggcatcacacgcgtctatggcctgatttttgataacatcagttacaccccccgtggctgtattggcatcacatgtgtctatgtggggtgatatgtcaggctcttctccgtcacaggaatcatcactccagctgctctccaacaggtgtgctgaggccatgggccacagagatttggtgtcggcagcatccacattctggaaggtcatggaatacagcaaacggttcagtttttcctgaagctgtttcacctgagctacgagatcgaccttcggcagctgacaatcttccagtactttttctttacccttgccgccgtcctccagactcaggcgcatttcatttttcaccaagagcagctccgactgcagctgcctctggcagacggtgagcactgacatcacgccttcttgcttgcagagaggtgcatccttcaacgtcaccaggacaggctgcagatcaccctgtgggtcagggacaaccggctccaaagcagcatcatgggaggcctccacgtcgccggtgacctgggccttggcgccaccatccatgcgaggctgtgggtgggccccgggcacccgtgtgtgagctgtggctctgcgggcctgccgcctgtccagctccacctggcacctcaggaaccgctggtgcagcacctgcagctggcggctgaggcgggcacactgcgctcggagccactgcagctcgggaggcgccgccccggctgccaggggctgctgctccagggcgcggcggatgcgggccaaggccaacaggacggcctccagctcggcagagtgggccgccttccgctggttcagagcgtcgatttctaaatttctctcggcaatcgtcgcttcctttgctttcagggccgcttcgaactcctggatccgggaggccatgtcttcgacctcagcctccctgagggctacattgcgctccagctcagccagctgtagctccgcagcctcctctgcgccctggaggcgctgctgcagggcctccagggcctggctgtgcctgcgctcctggtcagccagcagccggctcagggcctccttggcttccagcgcagcctcgagctcgccctgtagggcctgcccacgagggcccccggcctgggagcagagcagctcgctctgcagactgccagcctgactgtcgctgacttcgtgcaccacaggccccatgagggacagctcgtgctgcagcttctcaatgacttcatggagttgttcaatttcctctgctttctccttttgtaatcgtttctgattctcttgcagattttcaatagtggctttcagctcttcaatctcagaacttctggtatatatgaccttcaagctcgtgttctcttcctcaagttctctgaggctgacagcagtctggctgttctgcatgtccaattttaagttcagatgtagtatttcttcatttttactttctaagtcacctttcatcttttctagctgttcttttaagtccaaaacctcgctctcgcgccgcaggagtgctctctgtgtcacctctaactgtatttctggaccctcaggagggctgcccgaaggaggctcgggacatctgcctgcatctagtgtagactgcaacgtggacgccagaagcaagctactcatctgctgtttctttaacacctctttatcctgttccagccctttcacgatgtttttctgtttttccacttcttcctggagctgggccacttttttcctgatgttgatgttcatctcctccagacgtttaatttcttcttcctgcattaacacttgtctatctgccgactctttctgtatagccaattcattaaattcatccaacttttctctcaacttttgttgtaacaactcaacctctccatccagcggcgcctgctggctgtcgcgagggccccagggctgcggcttggccgcctggcggagctgcccctccagcctctgaatctcctgctggaactcctcgcgctcgtgctcccgctcggctgcctgctcatccatgaattgccgctggttgcgcaaatgcttgtccagagatgccacctgctgttccagggcagtgacggcctccgcctgcttggcacacccgcgatgctgagacagctgttcttctaactcagactccaaaatcttcatctgggagagcagggctgagcggtccttctcagcctgcttcctggtctccgactgttctttggtcagatcctccacttccttccggagagcagcttctctggcctcggcgtccgtggctgtggcctccccccgactccacagacgggtgcactcctccctcagcgccgcctgctcctgggccgcctgctgcagctgccgtctcaggctctccagctccagcaccagacggtgctcggaatcctccttcccggccagcacctccttcagatctgctgtctccaccttgaatccctcaagggtaccctgagtcttgtgcagctccagcgccagctctgcctttgctgcgctctcctccttcaaacactccagcagctcctggtgcttcctgacaacctgtgctgtctcctcattcttaaaactaaattctttttcaaaacgagaatgaatttggcgtgcttcttccagctgcctgctggagtccagggccatctccatgaggccgtccacggccaggctgaggctctggaagaccctccggatgggctgctcacactcccgcacactttctgggctcatgagaaagctttcacgcatgtggctgctaatttcagccacggaagacatctctgcacattcagacaaagttctgtccaactccgggagggccacatcagaccatgtctcctccagcgccggagctgtcgacagggccaggcctgcgcccgcgtcatccaggcagagccccacgcgctccccgatccggctcctcagggtgacggctgccctcagcgtctctccaaacaaacccagcagcctgcgcagggcgtcctggagggcccctctttcgctgtgggacaggttgacgtcggccttgagcatggagaggaggtttgcgccttcccggttctcccgctcccgcctctgctgcagcacctccaactcggagcggcactcttctatctcgtgacttaaggataaaacctggtctttcagctgctggacttggtgattcttcttttgaagctgcagagacaaagactctttctcctcttggtgaaaaggctgtgcctgtgcactctgaagccgaagtgtctcctctttttcatgcaaagcagttttcttttcacttccaaattcaccctggtgcactccctgcagctcgtgagccacggttccggcgagctctgtgctcacttcggttcgcaggtggtcccgcacagactgtagctccccttcgtgtttccgcttcagtttctccaactcttgagtcaaaatcgtttggtgaagagagtcctttttccacagttgttcctcaaagtctgctcgtaagagctctagggcctgcctgtgctcctcacggatggtctgaaattcagagaggtaacaggattccaaagaatcaaggctggacagatgtctggtctccagagcgccgaggtcggcagcgtgttttgtctgcagttcggccacacgtgcagccagcagagccccctgcttgctctctaaggaggctgtcagctcgcccaacgcggcctggtgtctggcctcgagctccgccgtcactgacaggagctgctgctggtgtctctcctggaggagctgcagctcacgggcatgctgctcctgggcctcctgcaggaaggcatcttgttccgcactgaatttctcggtgatctctttacgttcctctaaaaacctgctccgggccagcatcagctgcagggcgcagtcttccttcacgtggagcgcagcaagctccccgtcctgggctgtgggcggctcccgcccacactggctgcaatgcagggcgtcgtctgaagtgaggtcctgttccagctgctgcaggcggccctgctgctccgtcaaggacctctccagatccaggatctgggctgcctgttggtcctgaagctgcctcatttcagcttctcgaagctcaaacttgtttatgatggtctgtttctcggattcagccttttctctcagttcaagtagcatcaatgttaacttctcctcagcttcccgctgtagctcctccttcataactttccagtccgtttcttttctttggaattcctgtttcatcagctcagtcttttgcttagcattatttagttccttctggtggtcttcaattagattgtgttttaccttctccaaatcgtccttcagacgagtttcatgctgcaacttcccatacaaatttctattttctatttttaggagttcaatttcttctttgagctcagtctgaagaagcgaaagttgcaccttgtgctcagtttccagacccaagactctggctgcccgctctgtgtcggcctccaagtccccgtcctgcacaccctggagatgcacccagggaagctcttggctgtgcccttcagagggttccagacgccactcgtgtcccaatgctgaagtctctacgcagcatctgtctgagacatgcccctcgtgctggatgcagaggggagactccagcgcttccagctggtgcctgtggctttcttctaactccgcctggaagcgtggcaggctctccttatgtcgctcaggctcgagttcatcaacgtgatcttttcttcctttctcaggtttctcttctaaacccacacaggacaacccaacttccacagagtccagaagagcatcttccctcgccccctgcagcctctgctgtaacagggttaggtcttcttggtaagttttctcagcatcccttaacttcttttcaaaataaatcctcagttgctccagttcggactcatgctgggttttttctcgctgcttcagctgttctaaatcttccacacgagaggtgcgcgccaggagttgctcatgtagctcactcaattcctgtctactggtcctggcagaatcaagctgggaccacaagcgcctgatctcttcttgtgattgtgccttcaggtcttcatatgatgcttgaagattctctaactccagctgtttttctttctcgctctctttgaacttgaactccaagtcttctaaacaccggccgtgctcggactgcaggtcttcacgtaacttctcaatggctgcttgatgatgactctccaggttcctaagggcccgttcagcctggtttttgtcttgaaaaatcttctccaactcagctctctgttctgccaattctttctgaaactggttttgtaaatcctccatttctgattgatgctttgcagacagttctttgcgtagattttctaaacataaatctttttcagattcccaatcttccttcagggtctttactatctgggcgtttttctccatttctgattgtaacttctccttcagctcagctgcttcctgtccacacctgagcaccacctcctccttctcccgtgcgtgctgctccctgaggagctccagctcgtgctgctgcctgctctgtagcagggccagctcctgggcacgccggctgttgagcatctcccgcagctccgtcaatgccgtctccttctccttctggaggttggcctgtgtcagctccagctgcgccgtgtgcatgttgctcagactcaggcgcagcgcctccagctcaaggccatgcacggcctgactctgatgcaggccagcctcatcttcacggccgctctccaggtcagtaatggcaagttcacattcttgttcacactccagtgaagacacaaccttagtgaagggctggggaagagaggagtgacctgagtaaccttggaaaacagttgtgactggaaactttgtgaacatcccacgctgttctgctgggtggtcactgattgtgaagatcccacgctgttctggtgtgtggtcactgactgtgaacatcccacgctgttccggttggtggtcactgattgtgaacatcccacgctgttctggtgggtggtcactgactgtgaacatcccatgctgttctggtgggtggtcactgactgtgaacatcccacgctgttctggtgggtggtcaccgactgtgaacatcccatgctgttctggtgggtggtcactgactgtgaacatcccacactgctctggaggatggtcattgacttgcttctgctgcagctgttccaagtcctctctcttctctccatcacagtcctccggctgagctgcaaaggcccctcctgccccatcaggggtgtcgtcacatgatgtgcttttgcaaatgtcccctcctccacagagtgcgctgtcctccttggttaccggactctcctcctggacagacgcatcgacagccgagcccttcctcttcgccgtctttttctccgaatgcgaactgtcaccttttgtttttctctgtcggaagtgagcaagcttcgtcctcccggcctccacctttctgcgccgctgctcttgctcaacttccatctccctcagactccgcgcgggccgcccggcggtgacggggctgacacagagcagccttcgctctatttacactccctcccccgcgcttgggctcgccctccccccgc

SEQ ID NO: 9050 - RNA, 8674 nt, Homo sapiens
  source 1..8674: mol_type = other RNA
actgagcctctctctctccagagagcatctcagctctcgtttttgggtgtgcagggcttccaccgtcgacttcagtgtggcacttacctccttctctctcctgagcgcctcacagtgcttctgagcctcagcctcaagctgctgctgagaatgcagggcttgctgctgcaccttttcaagcatcgcttgcaagtccaccacccgggacttctcctccttcagcttctgcagcagagcgtgatgggcctgtgtgtcctggtgcacgcaagcctcctgtgtcctctggctcagctgctcggtcaggagccgctcgtgccgcaaggcctctgacagctccagggtgcggctcttctcagccgcaaggtccttctggagctcagagagctggctccgctcctgagccagcaaggcctcgcagcgtgagtgctcgatacgcagctccttctgcaggttgtccttggccgtctgctcgtgtttcagtgccacgcagagtcgactgctctgagcacgctgtgtctccaaagacgcccgcagctcctccagggccttggcactctggctctccctctgcaggtgccgcagctgctcctcctccagctggctctgcagggcacgccccttcccctgctcactctccagctcctgaagcgcggccttcagctcgttctccttactgctcagcatggatctcagctggaggacctcctgctgcacctcgcagagggaccgggacagctgttcgctcttctgcctgctctcacagaggtcggacttcaaatctcgcactacagtctgctccgccgccaggagcttctgcacgctgtttgccttctcttgctcttcactcagcgtcttctgcaagtcaccagcaatgcacttctcctgctctactttataagccagcagttcaacctgcctgcgcagctggtgctcctgctggctcccgcgcgcctctgcgcttgtcagcgccgtgcgcaagtgctgcagcttctcctggttctgcaggtgcgtcatgcgcagctgggcacgcagcgcctggatctcggacagcaggctgctccggtccggcaagcgaagatgctccagggacttttcctgcaggtctccctgctcacggatgatcttctccagcctttcgagcagggagctgtgaccccccagatctgagccactgagtcggggctgcagctcaaccccctgcatctcctgctctttttcaaaggcctcttgcacaacctgcagaaggtcccctctccaatcggggcacgcggtgggcacttcctgcgtctttcccccatggagcgagatgtcctgtatctcgtcttccttccggggtgggtgtggctcgccgcttgggggtgcaaggccttctgacagcgccaggatctggtggctctcgtcacgcaccatctgcagtaaagccttcacgtgcttcggacgcacttccttctccttcatggcttccggcagcggctgaaaccttccagagatggaagcaggggtcacaggaccagcagtttgagcctcagggcctcctgaccccgggctcagtcttgctccaaaacccgagccgtcacttttctcacttctatcagcttttccttctaatccaggaggaggtgaacttaatgtttcttgagaatcaaaggatgttgtgataaaatcttcgacatctttctccacagccgtcctctgcacatggtggtcgtcagccggcggagactcggcccactgcagtgccagcgctgctgcagacacgcctggggaacaaagcagccccggcccctgggtctgtggcagcgaggtgtccgccctgtcccccagggatgtgtcggcactgcacaggctcagggctcctgagtggggtgtcacggggaggctgggccagggctccagggtccagtccttcctgaggacctcaggggagctccaggaagacaggtccagcatcccgaccgggctcttccggggcccagcctctgcagtgtggctctggtggcgggagccaccaagtacgctggtcggtgaagaaagagacatgtcctgacattctgatttttcttgaatgggagaatctggcatttcatctggtatcaaggaatcccaatttttgataacatcagttacaccccctggggttgtattggcatcacacgcgtctatggcctgatttttgataacatcagttacaccccccgtggctgtattggcatcacatgtgtctatgtggggtgatatgtcaggctcttctccgtcacaggaatcatcactccagctgctctccaacaggtgtgctgaggccatgggccacagagatttggtgtcggcagcatccacattctggaaggtcatggaatacagcaaacggttcagtttttcctgaagctgtttcacctgagctacgagatcgaccttcggcagctgacaatcttccagtactttttctttacccttgccgccgtcctccagactcaggcgcatttcatttttcaccaagagcagctccgactgcagctgcctctggcagacggtgagcactgacatcacgccttcttgcttgcagagaggtgcatccttcaacgtcaccaggacaggctgcagatcaccctgtgggtcagggacaaccggctccaaagcagcatcatgggaggcctccacgtcgccggtgacctgggccttggcgccaccatccatgcgaggctgtgggtgggccccgggcacccgtgtgtgagctgtggctctgcgggcctgccgcctgtccagctccacctggcacctcaggaaccgctggtgcagcacctgcagctggcggctgaggcgggcacactgcgctcggagccactgcagctcgggaggcgccgccccggctgccaggggctgctgctccagggcgcggcggatgcgggccaaggccaacaggacggcctccagctcggcagagtgggccgccttccgctggttcagagcgtcgatttctaaatttctctcggcaatcgtcgcttcctttgctttcagggccgcttcgaactcctggatccgggaggccatgtcttcgacctcagcctccctgagggctacattgcgctccagctcagccagctgtagctccgcagcctcctctgcgccctggaggcgctgctgcagggcctccagggcctggctgtgcctgcgctcctggtcagccagcagccggctcagggcctccttggcttccagcgcagcctcgagctcgccctgtagggcctgcccacgagggcccccggcctgggagcagagcagctcgctctgcagactgccagcctgactgtcgctgacttcgtgcaccacaggccccatgagggacagctcgtgctgcagcttctcaatgacttcatggagttgttcaatttcctctgctttctccttttgtaatcgtttctgattctcttgcagattttcaatagtggctttcagctcttcaatctcagaacttctggtatatatgaccttcaagctcgtgttctcttcctcaagttctctgaggctgacagcagtctggctgttctgcatgtccaattttaagttcagatgtagtatttcttcatttttactttctaagtcacctttcatcttttctagctgttcttttaagtccaaaacctcgctctcgcgccgcaggagtgctctctgtgtcacctctaactgtatttctggaccctcaggagggctgcccgaaggaggctcgggacatctgcctgcatctagtgtagactgcaacgtggacgccagaagcaagctactcatctgctgtttctttaacacctctttatcctgttccagccctttcacgatgtttttctgtttttccacttcttcctggagctgggccacttttttcctgatgttgatgttcatctcctccagacgtttaatttcttcttcctgcattaacacttgtctatctgccgactctttctgtatagccaattcattaaattcatccaacttttctctcaacttttgttgtaacaactcaacctctccatccagcggcgcctgctggctgtcgcgagggccccagggctgcggcttggccgcctggcggagctgcccctccagcctctgaatctcctgctggaactcctcgcgctcgtgctcccgctcggctgcctgctcatccatgaattgccgctggttgcgcaaatgcttgtccagagatgccacctgctgttccagggcagtgacggcctccgcctgcttggcacacccgcgatgctgagacagctgttcttctaactcagactccaaaatcttcatctgggagagcagggctgagcggtccttctcagcctgcttcctggtctccgactgttctttggtcagatcctccacttccttccggagagcagcttctctggcctcggcgtccgtggctgtggcctccccccgactccacagacgggtgcactcctccctcagcgccgcctgctcctgggccgcctgctgcagctgccgtctcaggctctccagctccagcaccagacggtgctcggaatcctccttcccggccagcacctccttcagatctgctgtctccaccttgaatccctcaagggtaccctgagtcttgtgcagctccagcgccagctctgcctttgctgcgctctcctccttcaaacactccagcagctcctggtgcttcctgacaacctgtgctgtctcctcattcttaaaactaaattctttttcaaaacgagaatgaatttggcgtgcttcttccagctgcctgctggagtccagggccatctccatgaggccgtccacggccaggctgaggctctggaagaccctccggatgggctgctcacactcccgcacactttctgggctcatgagaaagctttcacgcatgtggctgctaatttcagccacggaagacatctctgcacattcagacaaagttctgtccaactccgggagggccacatcagaccatgtctcctccagcgccggagctgtcgacagggccaggcctgcgcccgcgtcatccaggcagagccccacgcgctccccgatccggctcctcagggtgacggctgccctcagcgtctctccaaacaaacccagcagcctgcgcagggcgtcctggagggcccctctttcgctgtgggacaggttgacgtcggccttgagcatggagaggaggtttgcgccttcccggttctcccgctcccgcctctgctgcagcacctccaactcggagcggcactcttctatctcgtgacttaaggataaaacctggtctttcagctgctggacttggtgattcttcttttgaagctgcagagacaaagactctttctcctcttggtgaaaaggctgtgcctgtgcactctgaagccgaagtgtctcctctttttcatgcaaagcagttttcttttcacttccaaattcaccctggtgcactccctgcagctcgtgagccacggttccggcgagctctgtgctcacttcggttcgcaggtggtcccgcacagactgtagctccccttcgtgtttccgcttcagtttctccaactcttgagtcaaaatcgtttggtgaagagagtcctttttccacagttgttcctcaaagtctgctcgtaagagctctagggcctgcctgtgctcctcacggatggtctgaaattcagagaggtaacaggattccaaagaatcaaggctggacagatgtctggtctccagagcgccgaggtcggcagcgtgttttgtctgcagttcggccacacgtgcagccagcagagccccctgcttgctctctaaggaggctgtcagctcgcccaacgcggcctggtgtctggcctcgagctccgccgtcactgacaggagctgctgctggtgtctctcctggaggagctgcagctcacgggcatgctgctcctgggcctcctgcaggaaggcatcttgttccgcactgaatttctcggtgatctctttacgttcctctaaaaacctgctccgggccagcatcagctgcagggcgcagtcttccttcacgtggagcgcagcaagctccccgtcctgggctgtgggcggctcccgcccacactggctgcaatgcagggcgtcgtctgaagtgaggtcctgttccagctgctgcaggcggccctgctgctccgtcaaggacctctccagatccaggatctgggctgcctgttggtcctgaagctgcctcatttcagcttctcgaagctcaaacttgtttatgatggtctgtttctcggattcagccttttctctcagttcaagtagcatcaatgttaacttctcctcagcttcccgctgtagctcctccttcataactttccagtccgtttcttttctttggaattcctgtttcatcagctcagtcttttgcttagcattatttagttccttctggtggtcttcaattagattgtgttttaccttctccaaatcgtccttcagacgagtttcatgctgcaacttcccatacaaatttctattttctatttttaggagttcaatttcttctttgagctcagtctgaagaagcgaaagttgcaccttgtgctcagtttccagacccaagactctggctgcccgctctgtgtcggcctccaagtccccgtcctgcacaccctggagatgcacccagggaagctcttggctgtgcccttcagagggttccagacgccactcgtgtcccaatgctgaagtctctacgcagcatctgtctgagacatgcccctcgtgctggatgcagaggggagactccagcgcttccagctggtgcctgtggctttcttctaactccgcctggaagcgtggcaggctctccttatgtcgctcaggctcgagttcatcaacgtgatcttttcttcctttctcaggtttctcttctaaacccacacaggacaacccaacttccacagagtccagaagagcatcttccctcgccccctgcagcctctgctgtaacagggttaggtcttcttggtaagttttctcagcatcccttaacttcttttcaaaataaatcctcagttgctccagttcggactcatgctgggttttttctcgctgcttcagctgttctaaatcttccacacgagaggtgcgcgccaggagttgctcatgtagctcactcaattcctgtctactggtcctggcagaatcaagctgggaccacaagcgcctgatctcttcttgtgattgtgccttcaggtcttcatatgatgcttgaagattctctaactccagctgtttttctttctcgctctctttgaacttgaactccaagtcttctaaacaccggccgtgctcggactgcaggtcttcacgtaacttctcaatggctgcttgatgatgactctccaggttcctaagggcccgttcagcctggtttttgtcttgaaaaatcttctccaactcagctctctgttctgccaattctttctgaaactggttttgtaaatcctccatttctgattgatgctttgcagacagttctttgcgtagattttctaaacataaatctttttcagattcccaatcttccttcagggtctttactatctgggcgtttttctccatttctgattgtaacttctccttcagctcagctgcttcctgtccacacctgagcaccacctcctccttctcccgtgcgtgctgctccctgaggagctccagctcgtgctgctgcctgctctgtagcagggccagctcctgggcacgccggctgttgagcatctcccgcagctccgtcaatgccgtctccttctccttctggaggttggcctgtgtcagctccagctgcgccgtgtgcatgttgctcagactcaggcgcagcgcctccagctcaaggccatgcacggcctgactctgatgcaggccagcctcatcttcacggccgctctccaggtcagtaatggcaagttcacattcttgttcacactcctttgtgaacatcccacgctgttctgctgggtggtcactgattgtgaagatcccacgctgttctggtgtgtggtcactgactgtgaacatcccacgctgttccggttggtggtcactgattgtgaacatcccacgctgttctggtgggtggtcactgactgtgaacatcccatgctgttctggtgggtggtcactgactgtgaacatcccacgctgttctggtgggtggtcaccgactgtgaacatcccatgctgttctggtgggtggtcactgactgtgaacatcccacactgctctggaggatggtcattgacttgcttctgctgcagctgttccaagtcctctctcttctctccatcacagtcctccggctgagctgcaaaggcccctcctgccccatcaggggtgtcgtcacatgatgtgcttttgcaaatgtcccctcctccacagagtgcgctgtcctccttggttaccggactctcctcctggacagacgcatcgacagccgagcccttcctcttcgccgtctttttctccgaatgcgaactgtcaccttttgtttttctctgtcggaagtgagcaagcttcgtcctcccggcctccacctttctgcgccgctgctcttgctcaacttccatctccctcagactccgcgcgggccgcccggcggtgacggggctgacacagagcagccttcgctctatttacact

SEQ ID NO: 9051 - RNA, 7822 nt, Homo sapiens
  source 1..7822: mol_type = other RNA
actgagcctctctctctccagagagcatctcagctctcgtttttgggtgtgcagggcttccaccgtcgacttcagtgtggcacttacctccttctctctcctgagcgcctcacagtgcttctgagcctcagcctcaagctgctgctgagaatgcagggcttgctgctgcaccttttcaagcatcgcttgcaagtccaccacccgggacttctcctccttcagcttctgcagcagagcgtgatgggcctgtgtgtcctggtgcacgcaagcctcctgtgtcctctggctcagctgctcggtcaggagccgctcgtgccgcaaggcctctgacagctccagggtgcggctcttctcagccgcaaggtccttctggagctcagagagctggctccgctcctgagccagcaaggcctcgcagcgtgagtgctcgatacgcagctccttctgcaggttgtccttggccgtctgctcgtgtttcagtgccacgcagagtcgactgctctgagcacgctgtgtctccaaagacgcccgcagctcctccagggccttggcactctggctctccctctgcaggtgccgcagctgctcctcctccagctggctctgcagggcacgccccttcccctgctcactctccagctcctgaagcgcggccttcagctcgttctccttactgctcagcatggatctcagctggaggacctcctgctgcacctcgcagagggaccgggacagctgttcgctcttctgcctgctctcacagaggtcggacttcaaatctcgcactacagtctgctccgccgccaggagcttctgcacgctgtttgccttctcttgctcttcactcagcgtcttctgcaagtcaccagcaatgcacttctcctgctctactttataagccagcagttcaacctgcctgcgcagctggtgctcctgctggctcccgcgcgcctctgcgcttgtcagcgccgtgcgcaagtgctgcagcttctcctggttctgcaggtgcgtcatgcgcagctgggcacgcagcgcctggatctcggacagcaggctgctccggtccggcaagcgaagatgctccagggacttttcctgcaggtctccctgctcacggatgatcttctccagcctttcgagcagggagctgtgaccccccagatctgagccactgagtcggggctgcagctcaaccccctgcatctcctgctctttttcaaaggcctcttgcacaacctgcagaaggtcccctctccaatcggggcacgcggtgggcacttcctgcgtctttcccccatggagcgagatgtcctgtatctcgtcttccttccggggtgggtgtggctcgccgcttgggggtgcaaggccttctgacagcgccaggatctggtggctctcgtcacgcaccatctgcagtaaagccttcacgtgcttcggacgcacttccttctccttcatggcttccggcagcggctgaaaccttccagagatggaagcaggggtcacaggaccagcagtttgagcctcagggcctcctgaccccgggctcagtcttgctccaaaacccgagccgtcacttttctcacttctatcagcttttccttctaatccaggaggaggtgaacttaatgtttcttgagaatcaaaggatgttgtgataaaatcttcgacatctttctccacagccgtcctctgcacatggtggtcgtcagccggcggagactcggcccactgcagtgccagcgctgctgcagacacgcctggggaacaaagcagccccggcccctgggtctgtggcagcgaggtgtccgccctgtcccccagggatgtgtcggcactgcacaggctcagggctcctgagtggggtgtcacggggaggctgggccagggctccagggtccagtccttcctgaggacctcaggggagctccaggaagacaggtccagcatcccgaccgggctcttccggggcccagcctctgcagtgtggctctggtggcgggagccaccaagtacgctggtcggtgaagaaagagacatgtcctgacattctgatttttcttgaatgggagaatctggcatttcatctggtatcaaggaatcccaatttttgataacatcagttacaccccctggggttgtattggcatcacacgcgtctatggcctgatttttgataacatcagttacaccccccgtggctgtattggcatcacatgtgtctatgtggggtgatatgtcaggctcttctccgtcacaggaatcatcactccagctgctctccaacaggtgtgctgaggccatgggccacagagatttggtgtcggcagcatccacattctggaaggtcatggaatacagcaaacggttcagtttttcctgaagctgtttcacctgagctacgagatcgaccttcggcagctgacaatcttccagtactttttctttacccttgccgccgtcctccagactcaggcgcatttcatttttcaccaagagcagctccgactgcagctgcctctggcagacggtgagcactgacatcacgccttcttgcttgcagagaggtgcatccttcaacgtcaccaggacaggctgcagatcaccctgtgggtcagggacaaccggctccaaagcagcatcatgggaggcctccacgtcgccggtgacctgggccttggcgccaccatccatgcgaggctgtgggtgggccccgggcacccgtgtgtgagctgtggctctgcgggcctgccgcctgtccagctccacctggcacctcaggaaccgctggtgcagcacctgcagctggcggctgaggcgggcacactgcgctcggagccactgcagctcgggaggcgccgccccggctgccaggggctgctgctccagggcgcggcggatgcgggccaaggccaacaggacggcctccagctcggcagagtgggccgccttccgctggttcagagcgtcgatttctaaatttctctcggcaatcgtcgcttcctttgctttcagggccgcttcgaactcctggatccgggaggccatgtcttcgacctcagcctccctgagggctacattgcgctccagctcagccagctgtagctccgcagcctcctctgcgccctggaggcgctgctgcagggcctccagggcctggctgtgcctgcgctcctggtcagccagcagccggctcagggcctccttggcttccagcgcagcctcgagctcgccctgtagggcctgcccacgagggcccccggcctgggagcagagcagctcgctctgcagactgccagcctgactgtcgctgacttcgtgcaccacaggccccatgagggacagctcgtgctgcagcttctcaatgacttcatggagttgttcaatttcctctgctttctccttttgtaatcgtttctgattctcttgcagattttcaatagtggctttcagctcttcaatctcagaacttctggtatatatgaccttcaagctcgtgttctcttcctcaagttctctgaggctgacagcagtctggctgttctgcatgtccaattttaagttcagatgtagtatttcttcatttttactttctaagtcacctttcatcttttctagctgttcttttaagtccaaaacctcgctctcgcgccgcaggagtgctctctgtgtcacctctaactgtatttctggaccctcaggagggctgcccgaaggaggctcgggacatctgcctgcatctagtgtagactgcaacgtggacgccagaagcaagctactcatctgctgtttctttaacacctctttatcctgttccagccctttcacgatgtttttctgtttttccacttcttcctggagctgggccacttttttcctgatgttgatgttcatctcctccagacgtttaatttcttcttcctgcattaacacttgtctatctgccgactctttctgtatagccaattcattaaattcatccaacttttctctcaacttttgttgtaacaactcaacctctccatccagcggcgcctgctggctgtcgcgagggccccagggctgcggcttggccgcctggcggagctgcccctccagcctctgaatctcctgctggaactcctcgcgctcgtgctcccgctcggctgcctgctcatccatgaattgccgctggttgcgcaaatgcttgtccagagatgccacctgctgttccagggcagtgacggcctccgcctgcttggcacacccgcgatgctgagacagctgttcttctaactcagactccaaaatcttcatctgggagagcagggctgagcggtccttctcagcctgcttcctggtctccgactgttctttggtcagatcctccacttccttccggagagctgagtccttgtgtgctgcagtgacagctgtgccagcttctctggcctcggcgtccgtggctgtggcctccccccgactccacagacgggtgcactcctccctcagcgccgcctgctcctgggccgcctgctgcagctgccgtctcaggctctccagctccagcaccagacggtgctcggaatcctccttcccggccagcacctccttcagatctgctgtctccaccttgaatccctcaagggtaccctgagtcttgtgcagctccagcgccagctctgcctttgctgcgctctcctccttcaaacactccagcagctcctggtgcttcctgacaacctgtgctgtctcctcattcttaaaactaaattctttttcaaaacgagaatgaatttggcgtgcttcttccagctgcctgctggagtccagggccatctccatgaggccgtccacggccaggctgaggctctggaagaccctccggatgggctgctcacactcccgcacactttctgggctcatgagaaagctttcacgcatgtggctgctaatttcagccacggaagacatctctgcacattcagacaaagttctgtccaactccgggagggccacatcagaccatgtctcctccagcgccggagctgtcgacagggccaggcctgcgcccgcgtcatccaggcagagccccacgcgctccccgatccggctcctcagggtgacggctgccctcagcgtctctccaaacaaacccagcagcctgcgcagggcgtcctggagggcccctctttcgctgtgggacaggttgacgtcggccttgagcatggagaggaggtttgcgccttcccggttctcccgctcccgcctctgctgcagcacctccaactcggagcggcactcttctatctcgtgacttaaggataaaacctggtctttcagctgctggacttggtgattcttcttttgaagctgcagagacaaagactctttctcctcttggtgaaaaggctgtgcctgtgcactctgaagccgaagtgtctcctctttttcatgcaaagcagttttcttttcacttccaaattcaccctggtgcactccctgcagctcgtgagccacggttccggcgagctctgtgctcacttcggttcgcaggtggtcccgcacagactgtagctccccttcgtgtttccgcttcagtttctccaactcttgagtcaaaatcgtttggtgaagagagtcctttttccacagttgttcctcaaagtctgctcgtaagagctctagggcctgcctgtgctcctcacggatggtctgaaattcagagaggtaacaggattccaaagaatcaaggctggacagatgtctggtctccagagcgccgaggtcggcagcgtgttttgtctgcagttcggccacacgtgcagccagcagagccccctgcttgctctctaaggaggctgtcagctcgcccaacgcggcctggtgtctggcctcgagctccgccgtcactgacaggagctgctgctggtgtctctcctggaggagctgcagctcacgggcatgctgctcctgggcctcctgcaggaaggcatcttgttccgcactgaatttctcggtgatctctttacgttcctctaaaaacctgctccgggccagcatcagctgcagggcgcagtcttccttcacgtggagcgcagcaagctccccgtcctgggctgtgggcggctcccgcccacactggctgcaatgcagggcgtcgtctgaagtgaggtcctgttccagctgctgcaggcggccctgctgctccgtcaaggacctctccagatccaggatctgggctgcctgttggtcctgaagctgcctcatttcagcttctcgaagctcaaacttgtttatgatggtctgtttctcggattcagccttttctctcagttcaagtagcatcaatgttaacttctcctcagcttcccgctgtagctcctccttcataactttccagtccgtttcttttctttggaattcctgtttcatcagctcagtcttttgcttagcattatttagttccttctggtggtcttcaattagattgtgttttaccttctccaaatcgtccttcagacgagtttcatgctgcaacttcccatacaaatttctattttctatttttaggagttcaatttcttctttgagctcagtctgaagaagcgaaagttgcaccttgtgctcagtttccagacccaagactctggctgcccgctctgtgtcggcctccaagtccccgtcctgcacaccctggagatgcacccagggaagctcttggctgtgcccttcagagggttccagacgccactcgtgtcccaatgctgaagtctctacgcagcatctgtctgagacatgcccctcgtgctggatgcagaggggagactccagcgcttccagctggtgcctgtggctttcttctaactccgcctggaagcgtggcaggctctccttatgtcgctcaggctcgagttcatcaacgtgatcttttcttcctttctcaggtttctcttctaaacccacacaggacaacccaacttccacagagtccagaagagcatcttccctcgccccctgcagcctctgctgtaacagggttaggtcttcttggtaagttttctcagcatcccttaacttcttttcaaaataaatcctcagttgctccagttcggactcatgctgggttttttctcgctgcttcagctgttctaaatcttccacacgagaggtgcgcgccaggagttgctcatgtagctcactcaattcctgtctactggtcctggcagaatcaagctgggaccacaagcgcctgatctcttcttgtgattgtgccttcaggtcttcatatgatgcttgaagattctctaactccagctgtttttctttctcgctctctttgaacttgaactccaagtcttctaaacaccggccgtgctcggactgcaggtcttcacgtaacttctcaatggctgcttgatgatgactctccaggttcctaagggcccgttcagcctggtttttgtcttgaaaaatcttctccaactcagctctctgttctgccaattctttctgaaactggttttgtaaatcctccatttctgattgatgctttgcagacagttctttgcgtagattttctaaacataaatctttttcagattcccaatcttccttcagggtcctgaaacagaccagcctctgcacaaggaccacccaccccgaaacagacgagcctctgcacgcaaggcctaatccacacagtcaccctcaaagcgttagtaatacatctccctataagtcccaggggccaatggcaactttgccaacctccacccaagggctgggctctgtcccaagtgttctgagaaatgggtctcactgcctgcgtcagaggagcagg

SEQ ID NO: 9052 - RNA, 8929 nt, Homo sapiens
  source 1..8929: mol_type = other RNA
actgagcctctctctctccagagagcatctcagctctcgtttttgggtgtgcagggcttccaccgtcgacttcagtgtggcacttacctccttctctctcctgagcgcctcacagtgcttctgagcctcagcctcaagctgctgctgagaatgcagggcttgctgctgcaccttttcaagcatcgcttgcaagtccaccacccgggacttctcctccttcagcttctgcagcagagcgtgatgggcctgtgtgtcctggtgcacgcaagcctcctgtgtcctctggctcagctgctcggtcaggagccgctcgtgccgcaaggcctctgacagctccagggtgcggctcttctcagccgcaaggtccttctggagctcagagagctggctccgctcctgagccagcaaggcctcgcagcgtgagtgctcgatacgcagctccttctgcaggttgtccttggccgtctgctcgtgtttcagtgccacgcagagtcgactgctctgagcacgctgtgtctccaaagacgcccgcagctcctccagggccttggcactctggctctccctctgcaggtgccgcagctgctcctcctccagctggctctgcagggcacgccccttcccctgctcactctccagctcctgaagcgcggccttcagctcgttctccttactgctcagcatggatctcagctggaggacctcctgctgcacctcgcagagggaccgggacagctgttcgctcttctgcctgctctcacagaggtcggacttcaaatctcgcactacagtctgctccgccgccaggagcttctgcacgctgtttgccttctcttgctcttcactcagcgtcttctgcaagtcaccagcaatgcacttctcctgctctactttataagccagcagttcaacctgcctgcgcagctggtgctcctgctggctcccgcgcgcctctgcgcttgtcagcgccgtgcgcaagtgctgcagcttctcctggttctgcaggtgcgtcatgcgcagctgggcacgcagcgcctggatctcggacagcaggctgctccggtccggcaagcgaagatgctccagggacttttcctgcaggtctccctgctcacggatgatcttctccagcctttcgagcagggagctgtgaccccccagatctgagccactgagtcggggctgcagctcaaccccctgcatctcctgctctttttcaaaggcctcttgcacaacctgcagaaggtcccctctccaatcggggcacgcggtgggcacttcctgcgtctttcccccatggagcgagatgtcctgtatctcgtcttccttccggggtgggtgtggctcgccgcttgggggtgcaaggccttctgacagcgccaggatctggtggctctcgtcacgcaccatctgcagtaaagccttcacgtgcttcggacgcacttccttctccttcatggcttccggcagcggctgaaaccttccagagatggaagcaggggtcacaggaccagcagtttgagcctcagggcctcctgaccccgggctcagtcttgctccaaaacccgagccgtcacttttctcacttctatcagcttttccttctaatccaggaggaggtgaacttaatgtttcttgagaatcaaaggatgttgtgataaaatcttcgacatctttctccacagccgtcctctgcacatggtggtcgtcagccggcggagactcggcccactgcagtgccagcgctgctgcagacacgcctggggaacaaagcagccccggcccctgggtctgtggcagcgaggtgtccgccctgtcccccagggatgtgtcggcactgcacaggctcagggctcctgagtggggtgtcacggggaggctgggccagggctccagggtccagtccttcctgaggacctcaggggagctccaggaagacaggtccagcatcccgaccgggctcttccggggcccagcctctgcagtgtggctctggtggcgggagccaccaagtacgctggtcggtgaagaaagagacatgtcctgacattctgatttttcttgaatgggagaatctggcatttcatctggtatcaaggaatcccaatttttgataacatcagttacaccccctggggttgtattggcatcacacgcgtctatggcctgatttttgataacatcagttacaccccccgtggctgtattggcatcacatgtgtctatgtggggtgatatgtcaggctcttctccgtcacaggaatcatcactccagctgctctccaacaggtgtgctgaggccatgggccacagagatttggtgtcggcagcatccacattctggaaggtcatggaatacagcaaacggttcagtttttcctgaagctgtttcacctgagctacgagatcgaccttcggcagctgacaatcttccagtactttttctttacccttgccgccgtcctccagactcaggcgcatttcatttttcaccaagagcagctccgactgcagctgcctctggcagacggtgagcactgacatcacgccttcttgcttgcagagaggtgcatccttcaacgtcaccaggacaggctgcagatcaccctgtgggtcagggacaaccggctccaaagcagcatcatgggaggcctccacgtcgccggtgacctgggccttggcgccaccatccatgcgaggctgtgggtgggccccgggcacccgtgtgtgagctgtggctctgcgggcctgccgcctgtccagctccacctggcacctcaggaaccgctggtgcagcacctgcagctggcggctgaggcgggcacactgcgctcggagccactgcagctcgggaggcgccgccccggctgccaggggctgctgctccagggcgcggcggatgcgggccaaggccaacaggacggcctccagctcggcagagtgggccgccttccgctggttcagagcgtcgatttctaaatttctctcggcaatcgtcgcttcctttgctttcagggccgcttcgaactcctggatccgggaggccatgtcttcgacctcagcctccctgagggctacattgcgctccagctcagccagctgtagctccgcagcctcctctgcgccctggaggcgctgctgcagggcctccagggcctggctgtgcctgcgctcctggtcagccagcagccggctcagggcctccttggcttccagcgcagcctcgagctcgccctgtagggcctgcccacgagggcccccggcctgggagcagagcagctcgctctgcagactgccagcctgactgtcgctgacttcgtgcaccacaggccccatgagggacagctcgtgctgcagcttctcaatgacttcatggagttgttcaatttcctctgctttctccttttgtaatcgtttctgattctcttgcagattttcaatagtggctttcagctcttcaatctcagaacttctggtatatatgaccttcaagctcgtgttctcttcctcaagttctctgaggctgacagcagtctggctgttctgcatgtccaattttaagttcagatgtagtatttcttcatttttactttctaagtcacctttcatcttttctagctgttcttttaagtccaaaacctcgctctcgcgccgcaggagtgctctctgtgtcacctctaactgtatttctggaccctcaggagggctgcccgaaggaggctcgggacatctgcctgcatctagtgtagactgcaacgtggacgccagaagcaagctactcatctgctgtttctttaacacctctttatcctgttccagccctttcacgatgtttttctgtttttccacttcttcctggagctgggccacttttttcctgatgttgatgttcatctcctccagacgtttaatttcttcttcctgcattaacacttgtctatctgccgactctttctgtatagccaattcattaaattcatccaacttttctctcaacttttgttgtaacaactcaacctctccatccagcggcgcctgctggctgtcgcgagggccccagggctgcggcttggccgcctggcggagctgcccctccagcctctgaatctcctgctggaactcctcgcgctcgtgctcccgctcggctgcctgctcatccatgaattgccgctggttgcgcaaatgcttgtccagagatgccacctgctgttccagggcagtgacggcctccgcctgcttggcacacccgcgatgctgagacagctgttcttctaactcagactccaaaatcttcatctgggagagcagggctgagcggtccttctcagcctgcttcctggtctccgactgttctttggtcagatcctccacttccttccggagagctgagtccttgtgtgctgcagtgacagctgtgccagcttctctggcctcggcgtccgtggctgtggcctccccccgactccacagacgggtgcactcctccctcagcgccgcctgctcctgggccgcctgctgcagctgccgtctcaggctctccagctccagcaccagacggtgctcggaatcctccttcccggccagcacctccttcagatctgctgtctccaccttgaatccctcaagggtaccctgagtcttgtgcagctccagcgccagctctgcctttgctgcgctctcctccttcaaacactccagcagctcctggtgcttcctgacaacctgtgctgtctcctcattcttaaaactaaattctttttcaaaacgagaatgaatttggcgtgcttcttccagctgcctgctggagtccagggccatctccatgaggccgtccacggccaggctgaggctctggaagaccctccggatgggctgctcacactcccgcacactttctgggctcatgagaaagctttcacgcatgtggctgctaatttcagccacggaagacatctctgcacattcagacaaagttctgtccaactccgggagggccacatcagaccatgtctcctccagcgccggagctgtcgacagggccaggcctgcgcccgcgtcatccaggcagagccccacgcgctccccgatccggctcctcagggtgacggctgccctcagcgtctctccaaacaaacccagcagcctgcgcagggcgtcctggagggcccctctttcgctgtgggacaggttgacgtcggccttgagcatggagaggaggtttgcgccttcccggttctcccgctcccgcctctgctgcagcacctccaactcggagcggcactcttctatctcgtgacttaaggataaaacctggtctttcagctgctggacttggtgattcttcttttgaagctgcagagacaaagactctttctcctcttggtgaaaaggctgtgcctgtgcactctgaagccgaagtgtctcctctttttcatgcaaagcagttttcttttcacttccaaattcaccctggtgcactccctgcagctcgtgagccacggttccggcgagctctgtgctcacttcggttcgcaggtggtcccgcacagactgtagctccccttcgtgtttccgcttcagtttctccaactcttgagtcaaaatcgtttggtgaagagagtcctttttccacagttgttcctcaaagtctgctcgtaagagctctagggcctgcctgtgctcctcacggatggtctgaaattcagagaggtaacaggattccaaagaatcaaggctggacagatgtctggtctccagagcgccgaggtcggcagcgtgttttgtctgcagttcggccacacgtgcagccagcagagccccctgcttgctctctaaggaggctgtcagctcgcccaacgcggcctggtgtctggcctcgagctccgccgtcactgacaggagctgctgctggtgtctctcctggaggagctgcagctcacgggcatgctgctcctgggcctcctgcaggaaggcatcttgttccgcactgaatttctcggtgatctctttacgttcctctaaaaacctgctccgggccagcatcagctgcagggcgcagtcttccttcacgtggagcgcagcaagctccccgtcctgggctgtgggcggctcccgcccacactggctgcaatgcagggcgtcgtctgaagtgaggtcctgttccagctgctgcaggcggccctgctgctccgtcaaggacctctccagatccaggatctgggctgcctgttggtcctgaagctgcctcatttcagcttctcgaagctcaaacttgtttatgatggtctgtttctcggattcagccttttctctcagttcaagtagcatcaatgttaacttctcctcagcttcccgctgtagctcctccttcataactttccagtccgtttcttttctttggaattcctgtttcatcagctcagtcttttgcttagcattatttagttccttctggtggtcttcaattagattgtgttttaccttctccaaatcgtccttcagacgagtttcatgctgcaacttcccatacaaatttctattttctatttttaggagttcaatttcttctttgagctcagtctgaagaagcgaaagttgcaccttgtgctcagtttccagacccaagactctggctgcccgctctgtgtcggcctccaagtccccgtcctgcacaccctggagatgcacccagggaagctcttggctgtgcccttcagagggttccagacgccactcgtgtcccaatgctgaagtctctacgcagcatctgtctgagacatgcccctcgtgctggatgcagaggggagactccagcgcttccagctggtgcctgtggctttcttctaactccgcctggaagcgtggcaggctctccttatgtcgctcaggctcgagttcatcaacgtgatcttttcttcctttctcaggtttctcttctaaacccacacaggacaacccaacttccacagagtccagaagagcatcttccctcgccccctgcagcctctgctgtaacagggttaggtcttcttggtaagttttctcagcatcccttaacttcttttcaaaataaatcctcagttgctccagttcggactcatgctgggttttttctcgctgcttcagctgttctaaatcttccacacgagaggtgcgcgccaggagttgctcatgtagctcactcaattcctgtctactggtcctggcagaatcaagctgggaccacaagcgcctgatctcttcttgtgattgtgccttcaggtcttcatatgatgcttgaagattctctaactccagctgtttttctttctcgctctctttgaacttgaactccaagtcttctaaacaccggccgtgctcggactgcaggtcttcacgtaacttctcaatggctgcttgatgatgactctccaggttcctaagggcccgttcagcctggtttttgtcttgaaaaatcttctccaactcagctctctgttctgccaattctttctgaaactggttttgtaaatcctccatttctgattgatgctttgcagacagttctttgcgtagattttctaaacataaatctttttcagattcccaatcttccttcagggtctttactatctgggcgtttttctccatttctgattgtaacttctccttcagctcagctgcttcctgtccacacctgagcaccacctcctccttctcccgtgcgtgctgctccctgaggagctccagctcgtgctgctgcctgctctgtagcagggccagctcctgggcacgccggctgttgagcatctcccgcagctccgtcaatgccgtctccttctccttctggaggttggcctgtgtcagctccagctgcgccgtgtgcatgttgctcagactcaggcgcagcgcctccagctcaaggccatgcacggcctgactctgatgcaggccagcctcatcttcacggccgctctccaggtcagtaatggcaagttcacattcttgttcacactcctttgtgaacatcccacgctgttctgctgggtggtcactgattgtgaagatcccacgctgttctggtgtgtggtcactgactgtgaacatcccacgctgttccggttggtggtcactgattgtgaacatcccacgctgttctggtgggtggtcactgactgtgaacatcccatgctgttctggtgggtggtcactgactgtgaacatcccacgctgttctggtgggtggtcaccgactgtgaacatcccatgctgttctggtgggtggtcactgactgtgaacatcccacactgctctggaggatggtcattgacttgcttctgctgcagctgttccaagtcctctctcttctctccatcacagtcctccggctgagctgcaaaggcccctcctgccccatcaggggtgtcgtcacatgatgtgcttttgcaaatgtcccctcctccacagagtgcgctgtcctccttggttaccggactctcctcctggacagacgcatcgacagccgagcccttcctcttcgccgtctttttctccgaatgcgaactgtcaccttttgtttttctctgtcggaagtgagcaagctcgcagaggccggcctgctcccgcggttccgcctcgcgctttcgggactccctttctcctgcccccgagtcatgggctctgcgcgctttattcccacgaaacctaggacagtggccatcaaaccgagcgctttttcacggagaaacccggggcgggagaaagacgggagcgcgtcccttgaaggcgcccggcgccagcgccgcgtgggttcccggcagcgtacgccaggcccggacgggcaggacgcgagcccaagggcgcgggaagaagacggcggccgggagcgccgcgggggcctttcacacagtaaggactgcaacgccgcgagaaacgcgcggggaaagcatc

SEQ ID NO: 9053 - RNA, 8741 nt, Homo sapiens
  source 1..8741: mol_type = other RNA
actgagcctctctctctccagagagcatctcagctctcgtttttgggtgtgcagggcttccaccgtcgacttcagtgtggcacttacctccttctctctcctgagcgcctcacagtgcttctgagcctcagcctcaagctgctgctgagaatgcagggcttgctgctgcaccttttcaagcatcgcttgcaagtccaccacccgggacttctcctccttcagcttctgcagcagagcgtgatgggcctgtgtgtcctggtgcacgcaagcctcctgtgtcctctggctcagctgctcggtcaggagccgctcgtgccgcaaggcctctgacagctccagggtgcggctcttctcagccgcaaggtccttctggagctcagagagctggctccgctcctgagccagcaaggcctcgcagcgtgagtgctcgatacgcagctccttctgcaggttgtccttggccgtctgctcgtgtttcagtgccacgcagagtcgactgctctgagcacgctgtgtctccaaagacgcccgcagctcctccagggccttggcactctggctctccctctgcaggtgccgcagctgctcctcctccagctggctctgcagggcacgccccttcccctgctcactctccagctcctgaagcgcggccttcagctcgttctccttactgctcagcatggatctcagctggaggacctcctgctgcacctcgcagagggaccgggacagctgttcgctcttctgcctgctctcacagaggtcggacttcaaatctcgcactacagtctgctccgccgccaggagcttctgcacgctgtttgccttctcttgctcttcactcagcgtcttctgcaagtcaccagcaatgcacttctcctgctctactttataagccagcagttcaacctgcctgcgcagctggtgctcctgctggctcccgcgcgcctctgcgcttgtcagcgccgtgcgcaagtgctgcagcttctcctggttctgcaggtgcgtcatgcgcagctgggcacgcagcgcctggatctcggacagcaggctgctccggtccggcaagcgaagatgctccagggacttttcctgcaggtctccctgctcacggatgatcttctccagcctttcgagcagggagctgtgaccccccagatctgagccactgagtcggggctgcagctcaaccccctgcatctcctgctctttttcaaaggcctcttgcacaacctgcagaaggtcccctctccaatcggggcacgcggtgggcacttcctgcgtctttcccccatggagcgagatgtcctgtatctcgtcttccttccggggtgggtgtggctcgccgcttgggggtgcaaggccttctgacagcgccaggatctggtggctctcgtcacgcaccatctgcagtaaagccttcacgtgcttcggacgcacttccttctccttcatggcttccggcagcggctgaaaccttccagagatggaagcaggggtcacaggaccagcagtttgagcctcagggcctcctgaccccgggctcagtcttgctccaaaacccgagccgtcacttttctcacttctatcagcttttccttctaatccaggaggaggtgaacttaatgtttcttgagaatcaaaggatgttgtgataaaatcttcgacatctttctccacagccgtcctctgcacatggtggtcgtcagccggcggagactcggcccactgcagtgccagcgctgctgcagacacgcctggggaacaaagcagccccggcccctgggtctgtggcagcgaggtgtccgccctgtcccccagggatgtgtcggcactgcacaggctcagggctcctgagtggggtgtcacggggaggctgggccagggctccagggtccagtccttcctgaggacctcaggggagctccaggaagacaggtccagcatcccgaccgggctcttccggggcccagcctctgcagtgtggctctggtggcgggagccaccaagtacgctggtcggtgaagaaagagacatgtcctgacattctgatttttcttgaatgggagaatctggcatttcatctggtatcaaggaatcccaatttttgataacatcagttacaccccctggggttgtattggcatcacacgcgtctatggcctgatttttgataacatcagttacaccccccgtggctgtattggcatcacatgtgtctatgtggggtgatatgtcaggctcttctccgtcacaggaatcatcactccagctgctctccaacaggtgtgctgaggccatgggccacagagatttggtgtcggcagcatccacattctggaaggtcatggaatacagcaaacggttcagtttttcctgaagctgtttcacctgagctacgagatcgaccttcggcagctgacaatcttccagtactttttctttacccttgccgccgtcctccagactcaggcgcatttcatttttcaccaagagcagctccgactgcagctgcctctggcagacggtgagcactgacatcacgccttcttgcttgcagagaggtgcatccttcaacgtcaccaggacaggctgcagatcaccctgtgggtcagggacaaccggctccaaagcagcatcatgggaggcctccacgtcgccggtgacctgggccttggcgccaccatccatgcgaggctgtgggtgggccccgggcacccgtgtgtgagctgtggctctgcgggcctgccgcctgtccagctccacctggcacctcaggaaccgctggtgcagcacctgcagctggcggctgaggcgggcacactgcgctcggagccactgcagctcgggaggcgccgccccggctgccaggggctgctgctccagggcgcggcggatgcgggccaaggccaacaggacggcctccagctcggcagagtgggccgccttccgctggttcagagcgtcgatttctaaatttctctcggcaatcgtcgcttcctttgctttcagggccgcttcgaactcctggatccgggaggccatgtcttcgacctcagcctccctgagggctacattgcgctccagctcagccagctgtagctccgcagcctcctctgcgccctggaggcgctgctgcagggcctccagggcctggctgtgcctgcgctcctggtcagccagcagccggctcagggcctccttggcttccagcgcagcctcgagctcgccctgtagggcctgcccacgagggcccccggcctgggagcagagcagctcgctctgcagactgccagcctgactgtcgctgacttcgtgcaccacaggccccatgagggacagctcgtgctgcagcttctcaatgacttcatggagttgttcaatttcctctgctttctccttttgtaatcgtttctgattctcttgcagattttcaatagtggctttcagctcttcaatctcagaacttctggtatatatgaccttcaagctcgtgttctcttcctcaagttctctgaggctgacagcagtctggctgttctgcatgtccaattttaagttcagatgtagtatttcttcatttttactttctaagtcacctttcatcttttctagctgttcttttaagtccaaaacctcgctctcgcgccgcaggagtgctctctgtgtcacctctaactgtatttctggaccctcaggagggctgcccgaaggaggctcgggacatctgcctgcatctagtgtagactgcaacgtggacgccagaagcaagctactcatctgctgtttctttaacacctctttatcctgttccagccctttcacgatgtttttctgtttttccacttcttcctggagctgggccacttttttcctgatgttgatgttcatctcctccagacgtttaatttcttcttcctgcattaacacttgtctatctgccgactctttctgtatagccaattcattaaattcatccaacttttctctcaacttttgttgtaacaactcaacctctccatccagcggcgcctgctggctgtcgcgagggccccagggctgcggcttggccgcctggcggagctgcccctccagcctctgaatctcctgctggaactcctcgcgctcgtgctcccgctcggctgcctgctcatccatgaattgccgctggttgcgcaaatgcttgtccagagatgccacctgctgttccagggcagtgacggcctccgcctgcttggcacacccgcgatgctgagacagctgttcttctaactcagactccaaaatcttcatctgggagagcagggctgagcggtccttctcagcctgcttcctggtctccgactgttctttggtcagatcctccacttccttccggagagctgagtccttgtgtgctgcagtgacagctgtgccagcttctctggcctcggcgtccgtggctgtggcctccccccgactccacagacgggtgcactcctccctcagcgccgcctgctcctgggccgcctgctgcagctgccgtctcaggctctccagctccagcaccagacggtgctcggaatcctccttcccggccagcacctccttcagatctgctgtctccaccttgaatccctcaagggtaccctgagtcttgtgcagctccagcgccagctctgcctttgctgcgctctcctccttcaaacactccagcagctcctggtgcttcctgacaacctgtgctgtctcctcattcttaaaactaaattctttttcaaaacgagaatgaatttggcgtgcttcttccagctgcctgctggagtccagggccatctccatgaggccgtccacggccaggctgaggctctggaagaccctccggatgggctgctcacactcccgcacactttctgggctcatgagaaagctttcacgcatgtggctgctaatttcagccacggaagacatctctgcacattcagacaaagttctgtccaactccgggagggccacatcagaccatgtctcctccagcgccggagctgtcgacagggccaggcctgcgcccgcgtcatccaggcagagccccacgcgctccccgatccggctcctcagggtgacggctgccctcagcgtctctccaaacaaacccagcagcctgcgcagggcgtcctggagggcccctctttcgctgtgggacaggttgacgtcggccttgagcatggagaggaggtttgcgccttcccggttctcccgctcccgcctctgctgcagcacctccaactcggagcggcactcttctatctcgtgacttaaggataaaacctggtctttcagctgctggacttggtgattcttcttttgaagctgcagagacaaagactctttctcctcttggtgaaaaggctgtgcctgtgcactctgaagccgaagtgtctcctctttttcatgcaaagcagttttcttttcacttccaaattcaccctggtgcactccctgcagctcgtgagccacggttccggcgagctctgtgctcacttcggttcgcaggtggtcccgcacagactgtagctccccttcgtgtttccgcttcagtttctccaactcttgagtcaaaatcgtttggtgaagagagtcctttttccacagttgttcctcaaagtctgctcgtaagagctctagggcctgcctgtgctcctcacggatggtctgaaattcagagaggtaacaggattccaaagaatcaaggctggacagatgtctggtctccagagcgccgaggtcggcagcgtgttttgtctgcagttcggccacacgtgcagccagcagagccccctgcttgctctctaaggaggctgtcagctcgcccaacgcggcctggtgtctggcctcgagctccgccgtcactgacaggagctgctgctggtgtctctcctggaggagctgcagctcacgggcatgctgctcctgggcctcctgcaggaaggcatcttgttccgcactgaatttctcggtgatctctttacgttcctctaaaaacctgctccgggccagcatcagctgcagggcgcagtcttccttcacgtggagcgcagcaagctccccgtcctgggctgtgggcggctcccgcccacactggctgcaatgcagggcgtcgtctgaagtgaggtcctgttccagctgctgcaggcggccctgctgctccgtcaaggacctctccagatccaggatctgggctgcctgttggtcctgaagctgcctcatttcagcttctcgaagctcaaacttgtttatgatggtctgtttctcggattcagccttttctctcagttcaagtagcatcaatgttaacttctcctcagcttcccgctgtagctcctccttcataactttccagtccgtttcttttctttggaattcctgtttcatcagctcagtcttttgcttagcattatttagttccttctggtggtcttcaattagattgtgttttaccttctccaaatcgtccttcagacgagtttcatgctgcaacttcccatacaaatttctattttctatttttaggagttcaatttcttctttgagctcagtctgaagaagcgaaagttgcaccttgtgctcagtttccagacccaagactctggctgcccgctctgtgtcggcctccaagtccccgtcctgcacaccctggagatgcacccagggaagctcttggctgtgcccttcagagggttccagacgccactcgtgtcccaatgctgaagtctctacgcagcatctgtctgagacatgcccctcgtgctggatgcagaggggagactccagcgcttccagctggtgcctgtggctttcttctaactccgcctggaagcgtggcaggctctccttatgtcgctcaggctcgagttcatcaacgtgatcttttcttcctttctcaggtttctcttctaaacccacacaggacaacccaacttccacagagtccagaagagcatcttccctcgccccctgcagcctctgctgtaacagggttaggtcttcttggtaagttttctcagcatcccttaacttcttttcaaaataaatcctcagttgctccagttcggactcatgctgggttttttctcgctgcttcagctgttctaaatcttccacacgagaggtgcgcgccaggagttgctcatgtagctcactcaattcctgtctactggtcctggcagaatcaagctgggaccacaagcgcctgatctcttcttgtgattgtgccttcaggtcttcatatgatgcttgaagattctctaactccagctgtttttctttctcgctctctttgaacttgaactccaagtcttctaaacaccggccgtgctcggactgcaggtcttcacgtaacttctcaatggctgcttgatgatgactctccaggttcctaagggcccgttcagcctggtttttgtcttgaaaaatcttctccaactcagctctctgttctgccaattctttctgaaactggttttgtaaatcctccatttctgattgatgctttgcagacagttctttgcgtagattttctaaacataaatctttttcagattcccaatcttccttcagggtctttactatctgggcgtttttctccatttctgattgtaacttctccttcagctcagctgcttcctgtccacacctgagcaccacctcctccttctcccgtgcgtgctgctccctgaggagctccagctcgtgctgctgcctgctctgtagcagggccagctcctgggcacgccggctgttgagcatctcccgcagctccgtcaatgccgtctccttctccttctggaggttggcctgtgtcagctccagctgcgccgtgtgcatgttgctcagactcaggcgcagcgcctccagctcaaggccatgcacggcctgactctgatgcaggccagcctcatcttcacggccgctctccaggtcagtaatggcaagttcacattcttgttcacactcctttgtgaacatcccacgctgttctgctgggtggtcactgattgtgaagatcccacgctgttctggtgtgtggtcactgactgtgaacatcccacgctgttccggttggtggtcactgattgtgaacatcccacgctgttctggtgggtggtcactgactgtgaacatcccatgctgttctggtgggtggtcactgactgtgaacatcccacgctgttctggtgggtggtcaccgactgtgaacatcccatgctgttctggtgggtggtcactgactgtgaacatcccacactgctctggaggatggtcattgacttgcttctgctgcagctgttccaagtcctctctcttctctccatcacagtcctccggctgagctgcaaaggcccctcctgccccatcaggggtgtcgtcacatgatgtgcttttgcaaatgtcccctcctccacagagtgcgctgtcctccttggttaccggactctcctcctggacagacgcatcgacagccgagcccttcctcttcgccgtctttttctccgaatgcgaactgtcaccttttgtttttctctgtcggaagtgagcaagcttcgtcctcccggcctccacctttctgcgccgctgctcttgctcaacttccatctccctcagactccgcgcgggccgcccggcggtgacggggctgacacagagcagccttcgctctatttacactccctcccccgcgcttgggctcgccctccccccgc

SEQ ID NO: 9054 - RNA, 8590 nt, Homo sapiens
  source 1..8590: mol_type = other RNA
actgagcctctctctctccagagagcatctcagctctcgtttttgggtgtgcagggcttccaccgtcgacttcagtgtggcacttacctccttctctctcctgagcgcctcacagtgcttctgagcctcagcctcaagctgctgctgagaatgcagggcttgctgctgcaccttttcaagcatcgcttgcaagtccaccacccgggacttctcctccttcagcttctgcagcagagcgtgatgggcctgtgtgtcctggtgcacgcaagcctcctgtgtcctctggctcagctgctcggtcaggagccgctcgtgccgcaaggcctctgacagctccagggtgcggctcttctcagccgcaaggtccttctggagctcagagagctggctccgctcctgagccagcaaggcctcgcagcgtgagtgctcgatacgcagctccttctgcaggttgtccttggccgtctgctcgtgtttcagtgccacgcagagtcgactgctctgagcacgctgtgtctccaaagacgcccgcagctcctccagggccttggcactctggctctccctctgcaggtgccgcagctgctcctcctccagctggctctgcagggcacgccccttcccctgctcactctccagctcctgaagcgcggccttcagctcgttctccttactgctcagcatggatctcagctggaggacctcctgctgcacctcgcagagggaccgggacagctgttcgctcttctgcctgctctcacagaggtcggacttcaaatctcgcactacagtctgctccgccgccaggagcttctgcacgctgtttgccttctcttgctcttcactcagcgtcttctgcaagtcaccagcaatgcacttctcctgctctactttataagccagcagttcaacctgcctgcgcagctggtgctcctgctggctcccgcgcgcctctgcgcttgtcagcgccgtgcgcaagtgctgcagcttctcctggttctgcaggtgcgtcatgcgcagctgggcacgcagcgcctggatctcggacagcaggctgctccggtccggcaagcgaagatgctccagggacttttcctgcaggtctccctgctcacggatgatcttctccagcctttcgagcagggagctgtgaccccccagatctgagccactgagtcggggctgcagctcaaccccctgcatctcctgctctttttcaaaggcctcttgcacaacctgcagaaggtcccctctccaatcggggcacgcggtgggcacttcctgcgtctttcccccatggagcgagatgtcctgtatctcgtcttccttccggggtgggtgtggctcgccgcttgggggtgcaaggccttctgacagcgccaggatctggtggctctcgtcacgcaccatctgcagtaaagccttcacgtgcttcggacgcacttccttctccttcatggcttccggcagcggctgaaaccttccagagatggaagcaggggtcacaggaccagcagtttgagcctcagggcctcctgaccccgggctcagtcttgctccaaaacccgagccgtcacttttctcacttctatcagcttttccttctaatccaggaggaggtgaacttaatgtttcttgagaatcaaaggatgttgtgataaaatcttcgacatctttctccacagccgtcctctgcacatggtggtcgtcagccggcggagactcggcccactgcagtgccagcgctgctgcagacacgcctggggaacaaagcagccccggcccctgggtctgtggcagcgaggtgtccgccctgtcccccagggatgtgtcggcactgcacaggctcagggctcctgagtggggtgtcacggggaggctgggccagggctccagggtccagtccttcctgaggacctcaggggagctccaggaagacaggtccagcatcccgaccgggctcttccggggcccagcctctgcagtgtggctctggtggcgggagccaccaagtacgctggtcggtgaagaaagagacatgtcctgacattctgatttttcttgaatgggagaatctggcatttcatctggtatcaaggaatcccaatttttgataacatcagttacaccccctggggttgtattggcatcacacgcgtctatggcctgatttttgataacatcagttacaccccccgtggctgtattggcatcacatgtgtctatgtggggtgatatgtcaggctcttctccgtcacaggaatcatcactccagctgctctccaacaggtgtgctgaggccatgggccacagagatttggtgtcggcagcatccacattctggaaggtcatggaatacagcaaacggttcagtttttcctgaagctgtttcacctgagctacgagatcgaccttcggcagctgacaatcttccagtactttttctttacccttgccgccgtcctccagactcaggcgcatttcatttttcaccaagagcagctccgactgcagctgcctctggcagacggtgagcactgacatcacgccttcttgcttgcagagaggtgcatccttcaacgtcaccaggacaggctgcagatcaccctgtgggtcagggacaaccggctccaaagcagcatcatgggaggcctccacgtcgccggtgacctgggccttggcgccaccatccatgcgaggctgtgggtgggccccgggcacccgtgtgtgagctgtggctctgcgggcctgccgcctgtccagctccacctggcacctcaggaaccgctggtgcagcacctgcagctggcggctgaggcgggcacactgcgctcggagccactgcagctcgggaggcgccgccccggctgccaggggctgctgctccagggcgcggcggatgcgggccaaggccaacaggacggcctccagctcggcagagtgggccgccttccgctggttcagagcgtcgatttctaaatttctctcggcaatcgtcgcttcctttgctttcagggccgcttcgaactcctggatccgggaggccatgtcttcgacctcagcctccctgagggctacattgcgctccagctcagccagctgtagctccgcagcctcctctgcgccctggaggcgctgctgcagggcctccagggcctggctgtgcctgcgctcctggtcagccagcagccggctcagggcctccttggcttccagcgcagcctcgagctcgccctgtagggcctgcccacgagggcccccggcctgggagcagagcagctcgctctgcagactgccagcctgactgtcgctgacttcgtgcaccacaggccccatgagggacagctcgtgctgcagcttctcaatgacttcatggagttgttcaatttcctctgctttctccttttgtaatcgtttctgattctcttgcagattttcaatagtggctttcagctcttcaatctcagaacttctggtatatatgaccttcaagctcgtgttctcttcctcaagttctctgaggctgacagcagtctggctgttctgcatgtccaattttaagttcagatgtagtatttcttcatttttactttctaagtcacctttcatcttttctagctgttcttttaagtccaaaacctcgctctcgcgccgcaggagtgctctctgtgtcacctctaactgtatttctggaccctcaggagggctgcccgaaggaggctcgggacatctgcctgcatctagtgtagactgcaacgtggacgccagaagcaagctactcatctgctgtttctttaacacctctttatcctgttccagccctttcacgatgtttttctgtttttccacttcttcctggagctgggccacttttttcctgatgttgatgttcatctcctccagacgtttaatttcttcttcctgcattaacacttgtctatctgccgactctttctgtatagccaattcattaaattcatccaacttttctctcaacttttgttgtaacaactcaacctctccatccagcggcgcctgctggctgtcgcgagggccccagggctgcggcttggccgcctggcggagctgcccctccagcctctgaatctcctgctggaactcctcgcgctcgtgctcccgctcggctgcctgctcatccatgaattgccgctggttgcgcaaatgcttgtccagagatgccacctgctgttccagggcagtgacggcctccgcctgcttggcacacccgcgatgctgagacagctgttcttctaactcagactccaaaatcttcatctgggagagcagggctgagcggtccttctcagcctgcttcctggtctccgactgttctttggtcagatcctccacttccttccggagagctgagtccttgtgtgctgcagtgacagctgtgccagcttctctggcctcggcgtccgtggctgtggcctccccccgactccacagacgggtgcactcctccctcagcgccgcctgctcctgggccgcctgctgcagctgccgtctcaggctctccagctccagcaccagacggtgctcggaatcctccttcccggccagcacctccttcagatctgctgtctccaccttgaatccctcaagggtaccctgagtcttgtgcagctccagcgccagctctgcctttgctgcgctctcctccttcaaacactccagcagctcctggtgcttcctgacaacctgtgctgtctcctcattcttaaaactaaattctttttcaaaacgagaatgaatttggcgtgcttcttccagctgcctgctggagtccagggccatctccatgaggccgtccacggccaggctgaggctctggaagaccctccggatgggctgctcacactcccgcacactttctgggctcatgagaaagctttcacgcatgtggctgctaatttcagccacggaagacatctctgcacattcagacaaagttctgtccaactccgggagggccacatcagaccatgtctcctccagcgccggagctgtcgacagggccaggcctgcgcccgcgtcatccaggcagagccccacgcgctccccgatccggctcctcagggtgacggctgccctcagcgtctctccaaacaaacccagcagcctgcgcagggcgtcctggagggcccctctttcgctgtgggacaggttgacgtcggccttgagcatggagaggaggtttgcgccttcccggttctcccgctcccgcctctgctgcagcacctccaactcggagcggcactcttctatctcgtgacttaaggataaaacctggtctttcagctgctggacttggtgattcttcttttgaagctgcagagacaaagactctttctcctcttggtgaaaaggctgtgcctgtgcactctgaagccgaagtgtctcctctttttcatgcaaagcagttttcttttcacttccaaattcaccctggtgcactccctgcagctcgtgagccacggttccggcgagctctgtgctcacttcggttcgcaggtggtcccgcacagactgtagctccccttcgtgtttccgcttcagtttctccaactcttgagtcaaaatcgtttggtgaagagagtcctttttccacagttgttcctcaaagtctgctcgtaagagctctagggcctgcctgtgctcctcacggatggtctgaaattcagagaggtaacaggattccaaagaatcaaggctggacagatgtctggtctccagagcgccgaggtcggcagcgtgttttgtctgcagttcggccacacgtgcagccagcagagccccctgcttgctctctaaggaggctgtcagctcgcccaacgcggcctggtgtctggcctcgagctccgccgtcactgacaggagctgctgctggtgtctctcctggaggagctgcagctcacgggcatgctgctcctgggcctcctgcaggaaggcatcttgttccgcactgaatttctcggtgatctctttacgttcctctaaaaacctgctccgggccagcatcagctgcagggcgcagtcttccttcacgtggagcgcagcaagctccccgtcctgggctgtgggcggctcccgcccacactggctgcaatgcagggcgtcgtctgaagtgaggtcctgttccagctgctgcaggcggccctgctgctccgtcaaggacctctccagatccaggatctgggctgcctgttggtcctgaagctgcctcatttcagcttctcgaagctcaaacttgtttatgatggtctgtttctcggattcagccttttctctcagttcaagtagcatcaatgttaacttctcctcagcttcccgctgtagctcctccttcataactttccagtccgtttcttttctttggaattcctgtttcatcagctcagtcttttgcttagcattatttagttccttctggtggtcttcaattagattgtgttttaccttctccaaatcgtccttcagacgagtttcatgctgcaacttcccatacaaatttctattttctatttttaggagttcaatttcttctttgagctcagtctgaagaagcgaaagttgcaccttgtgctcagtttccagacccaagactctggctgcccgctctgtgtcggcctccaagtccccgtcctgcacaccctggagatgcacccagggaagctcttggctgtgcccttcagagggttccagacgccactcgtgtcccaatgctgaagtctctacgcagcatctgtctgagacatgcccctcgtgctggatgcagaggggagactccagcgcttccagctggtgcctgtggctttcttctaactccgcctggaagcgtggcaggctctccttatgtcgctcaggctcgagttcatcaacgtgatcttttcttcctttctcaggtttctcttctaaacccacacaggacaacccaacttccacagagtccagaagagcatcttccctcgccccctgcagcctctgctgtaacagggttaggtcttcttggtaagttttctcagcatcccttaacttcttttcaaaataaatcctcagttgctccagttcggactcatgctgggttttttctcgctgcttcagctgttctaaatcttccacacgagaggtgcgcgccaggagttgctcatgtagctctccagctgtttttctttctcgctctctttgaacttgaactccaagtcttctaaacaccggccgtgctcggactgcaggtcttcacgtaacttctcaatggctgcttgatgatgactctccaggttcctaagggcccgttcagcctggtttttgtcttgaaaaatcttctccaactcagctctctgttctgccaattctttctgaaactggttttgtaaatcctccatttctgattgatgctttgcagacagttctttgcgtagattttctaaacataaatctttttcagattcccaatcttccttcagggtctttactatctgggcgtttttctccatttctgattgtaacttctccttcagctcagctgcttcctgtccacacctgagcaccacctcctccttctcccgtgcgtgctgctccctgaggagctccagctcgtgctgctgcctgctctgtagcagggccagctcctgggcacgccggctgttgagcatctcccgcagctccgtcaatgccgtctccttctccttctggaggttggcctgtgtcagctccagctgcgccgtgtgcatgttgctcagactcaggcgcagcgcctccagctcaaggccatgcacggcctgactctgatgcaggccagcctcatcttcacggccgctctccaggtcagtaatggcaagttcacattcttgttcacactcctttgtgaacatcccacgctgttctgctgggtggtcactgattgtgaagatcccacgctgttctggtgtgtggtcactgactgtgaacatcccacgctgttccggttggtggtcactgattgtgaacatcccacgctgttctggtgggtggtcactgactgtgaacatcccatgctgttctggtgggtggtcactgactgtgaacatcccacgctgttctggtgggtggtcaccgactgtgaacatcccatgctgttctggtgggtggtcactgactgtgaacatcccacactgctctggaggatggtcattgacttgcttctgctgcagctgttccaagtcctctctcttctctccatcacagtcctccggctgagctgcaaaggcccctcctgccccatcaggggtgtcgtcacatgatgtgcttttgcaaatgtcccctcctccacagagtgcgctgtcctccttggttaccggactctcctcctggacagacgcatcgacagccgagcccttcctcttcgccgtctttttctccgaatgcgaactgtcaccttttgtttttctctgtcggaagtgagcaagcttcgtcctcccggcctccacctttctgcgccgctgctcttgctcaacttccatctccctcagactccgcgcgggccgcccggcggtgacggggctgacacagagcagccttcgctctattt

SEQ ID NO: 9055 - RNA, 14991 nt, Homo sapiens
  source 1..14991: mol_type = other RNA
actgagcctctctctctccagagctcattgggctttttgttgcttagttagatgagccatagacaaggagtttgagacctgggttttagcaactgctctgctaaaactggctgatcttgtggaagataaacctcattgagtcttagtttgtgctttttttaaagtgagatatttagttagactagtgattttcaaactctttttcctagtagcaagactctttgtacgaagaaaatcttatctggatgcccaacccagacaagagaggttaagagtcattctggttgactttgaaggtggactgtcttttctcccattgtggccatagtgaaagtgactctgtctaaaatttagtgtattttttccccccaaagatggataatgtgttaatgggacgatgtgagaaggataagaggtaaggatgtgggagtgagcaaggtgacagatcataggctatgctttttcatataaaaaatgaagatgggtattacagaagatattactaaattgtttctctgaaaagtcttataacttatgacatgaaactacattaaattatatgtgtcaacttcaaaacattacagtacctgaagtggacactgctttggctgtatgaccccagtaaggtagggtcagatgggcatctaggggactggcttttcctgcttatctaagtgatagaagttttcactgttaaaacttcattttattgctcttatttttgtcacaagtccttatgagcttggttgggtgaagggtcacccagaaaagaaccagcttccactttctttaattatgcaaactagagctaggtgactgagaacttgcttttggtctgcaagacatagggagttttgcaagccccaagggagtccagaatttcctgaacatgttgcaaggtggctggatggctttcttctgaagtcatgcaatattgtccttcactttggttatgactgcagaggtgctgggaagcaaaatgaaaactatcaccttgaagcaggcttttcttcataggccccagaggtgaggccagctcatttaaagggaatggcttgtgctgctgctttcatctaaaggtattttgatccaattccacctcccagctcctttattggtaatgttttccaaaacacagtatttttgctgagggaaggacaggcaaaggcctgaacatttagagagtagaaaactggctgggtgtggaccttttacaaaagttcatattttgctagtttaatttggaaaaggacacatgaattctcacagaaaatgagctttattggggaacaatacatttcatgaaggcatttctttatcaggaatcacacaggcagccccacgcagtcactgccccacaccttatccttcagcttgtgctgcacaggagaggagtggctgggattcctgactagggctttgatgagagtgcatgcacactggagcatgcttcttggcctggatggcaaagtcccaggagccagtcctaactcagactctggcctgcctaggtacatttcagatgaaagtcacccctgctccttgccccaccctcagtccaacaaaaatgtgcttctagaaatgcttacttttctttttctacgaagggcttataatgtgaggctactaaagattttcagatttcagaatagtaccacttaccttgggctaggttaattttttagagaattgatcttgtcccctaatgagtaggaagatcaactggtttttggacatgactataagcagaagatgctaaataataccttaaaaagactccactggccaggtgcggtggttcactcctgtaaacattttttaatttttgtgggtacatagtagatgtatatatttatgggttacatgaaatattttggtacaggcatgcaatgtgtaataatcacatcaggataaatagggtttccatcatcttaagcacttatcctttgtgttacaaacaatccagttatactcttcagttattttaaaattttattttttgagacagtctcactctattgcctaggctggagtgcagtgccacaatcatggctcactgaagccttgaccgcctggtctcaggtgatcttcaccctcctgagtagctgggactataggcgtgtgccaccatgcccggctaattgtttacttttttgtagagatggggtctccctatgttgcccaggctggtctcaaactcctgggctcaagtcatcctcccacctcagtctcccaaagtgctgggattacaggcgtgagccaccgtgcccggccagggagctctttcagattggctcctgtgtctgtctgacatgcttctatccttttgtttttgagcacttgcttagtttctggtactacaagatgctccaggcttatcttgcatttttttggctctagccttagaacctagctattttctcaagaagcctgggttcttttctattggaaaatatttagaaaccaaaatccagcacagtactttgaactgaattctgcttcagtcctcccaaactaacataaacttggcagaagtgtatgggaggcagatgcagcaccctcccaaagcagctggccctgtggtgacttggtggcagttgtccacttggatccttagtttctatactgagctactggctcctcacctgaggtctctagacttgtagggcatgtgagataactgaagagatatctctgggcacagagagggaagaagtggagatacagcagcttccctcattttttaatttttaatttttgagacagtgtcttgctctgtcacccaggctggagtgcagtggtgcaatcttggctccctacaacctctgcctcctgggctcaagtgatcctcccacctctgactcctgagtagctgggactccaggcatacaccgccatgcctggctaattttttttatttttggtggagacagggttttgctatgttgcccaagttggtctcaaactcctggactcaagcaatcagcccatcttggcttcccaaagtgctgggattacaggtgtgagcccctgtgcctggctagcttctttttctctttaccctaggtcactaggtcagagagagagaggccctgttataatctttgacttttaatagctttattaaggtataatttatacacataaactttacctgttttaagtgcataaatcaattatttttaaagtttataaagttgtgcaaaaatggctgggtgtggtggctcacgcctgtaatcccagcgctttgggaggccgaggcaggaggatcacctgaggtcaggagttcgagaccagcctgaccaacctggagaaaacctgtctctactaaaaatacaaaattagccgggcatggtggcacatgcctgtaatcccagctactcaggaagctgaggcaggagaaatgcttcaacccaggaggcggaggttgtggtgagctgagatcgcgccattgcactccagcctgggcaacaagagtgaaactccatctcacacacacacacacacacacacataaaagttgtgcaaaaattacaacttagttttggaacatttttgtcacccccaaaagatcccttgtgcccatctgcaggcaatccatgttttcacatcagacccatgcaactgctaatttagtatatgccttttctggactgtaaatggaaacataccatatgtgggatattgcatcagacttctttcactaagcataatgttttgagatgcatccatattgtagcctatatcactactccattgtatacatatatcatttaaagaaatccaccagttaaaaaaaaaaagaaaaagaaataatctgggtatgttggtgcctgcctgcagtcccagttactgaggaggctgaggcaggaggattgtttgagcccaggagtttgacttcagagtatgcaacatagtgaggcctcatctcttaaaaaaaaaaaaaaaatccagtagttgatggtcatttggtttccactttttgactaatatgaatgataatgctatgaacatttgcctacgagtcttgatgtgaacacatttccacttctcttctcatggaatagcaggatcatatggtaaacttatgtttatctttttaagaaactgccaaactgttttccaaagtggctgcaccattttacattcccaccagcaatgcattagggctccagtttctccacatcatcaccaacacatatctttgtctgtcttttttattatagtcattttagtgggtccaaaatggtatctaattttgcttttaacttgtattttcctaatgactagtgatagtacacatctcttcatatgctaagcaatttgtatatctttgctgaaatatctattcaaacattttgtccatttttaagttgtctgccttatttttgagttttaagaattctttacatagtctagatacaagtcctctatcagatacttattatggtttgaaaatattttctcccagtctgtgatttttcaattaatttttttttttttttttttttttgagacagggtctcactctgtcacccaggctctagtgcggtggtgtgatcttggctcactgcaacctctgcctcccagggtcaagagatcctcccacctcagccttctgagtagccaggactacaggagcacgccaccatgcctggttaatttttgtattttttgtggagatggcattttgctctgttgtccagtctggtctcaaattcctgagctcaagtggtccaccctccttggcttccgaaagtgcagggatttcagatgtgaaccacctccccgggccaattaattttcttaatagttttttgaaacaaaattttatattttaatgaagtccaatttattaatattttcttttatgaattgtgctattagtgtcttaagaattcttcctaaaccaaggtcatctaggttttctcccatgttttcttctacatgttttatagttttagctcttacatgtaggtgtgtgatcaattttgagtttatttttgcatatggtaggaggtaagaatctaaattaatttcttctgcatttgatatccaaatatcctagcactatttgttgaaaagaccatcttttctccataatttcattgggatttttgtcaaaacttaattgatcataaatgtgaaggtttattcctggactctgttccactgatctgtatgcctatctttatatcagtaccacactgtcttgattaatgtagctttgtagtaagttctggatcagaattatttcttcattttcagaattattttggctattctgaatcctttatgttttcatacagattttaagattggcttgtcaatttttcaaaaaagcctgctgtgattttgatagggattgcattgtagattaatttggggagaactgctatcttaacaacatttgatcttccaattcatgaacatggattgtgtctacatttcttgataccttctttaatctctctgaatttttctttttctttttttgagacagggtcttgctctgttgcccaggctggagtgcactggcacagtcacagctaactgcagcctcaacctcccaagctcaggcaatcctcccaatgtagcctctcaagtagctgggactacaggtgtgcagcaccatgcctggctagttttttaaaatttaataattattttttttattatactttaagttctgggttacatgtgcagaacatgtagttttgttacataggtatacacatgccatggtggtttgctgcacccaccaacctgtcacctacattaggtatttctcctaatgttatccctcccttagccccccaccccccacaggccctggtgtgtgatgttaccctccctgtgtccatgtgttctcattgtttaactcccacttatgagtgagaacatgcgttgtttggttttctgatcttgtgatagtttgctgagaatgatggtttccggctttatccatgtccctgcaaaggacatgaactcatccttttttatggctgcatagtattccatggtatacatgtgccacattttcttaatccagtctatcattgacgggcatttgggttggtttcaaatctttgctattgtgaatagtgcagcaataaacatacgtgtgcatgtgtctttattgtagaatgatttataatcttttgggtatatgcccaatagtgggattgctgggtcaaatggtatttccagttctagatccttgaggagtcgtcacactgacttccacaatggtcggactaatttgcactcccaccaacagtgtaaaagcgttccaatttttccacaacctctccagcatctattgtttcctgatttttaatgatcgccattctaactggcatgagatggtatctcactgtggttttgattttcatttctctaatgactagtgatgatgagcattttttcatatgtctgttggctgcataaatgtcttcttttgagaagtatctgttcatatcctttgcccattttttgatggggttgtttgcttttttcttgtaaatttgtttaagttctttgtagattctggatattagccctttgtcagatggatatattgcaaaaatgttctcccattctgtaggttgcctgttcactctgatgatagtttattttgctgtgcagaagctctttaattagaacccatttgtcaattttggcttttgttgccattgcttttggtgttttagacatgaagtctttgcccatgcctatgtcctgaatggtattgcccaggttttcttctaggatttttatggtcctaggtcttacgtttaagtctttgttccatcttgagttgatttttgtataaggtgtaaggaaagggtccagttacagttttctgcatatggctagcccgttttcccaacaccatttattaaatagggaatcttttccccattgcttgtgtgtgtcaggtttgtcaaagatcagatggtggtagacgtgtggtgttatttctgaggcctccattctgttccattcgtctgcatatctgtttttgtaccagtgccatgctgttttggttactgtaggcttgtagtaaagtttgaagtcaggtagtgtgatgcctccagctttgttcttcttgcccaggattgtcttggctaggtgggctcttttttggttccatatgaatcttaaagtagttttttccaattctgtgaagaaagttagtggtagcttgatggggatagcattgaatctataaatcagtttgggcaacaaggccattgtcatgatattgattcttcctatccatgagcatggaatgtttttccatttgtttgtgtcctctcttatttccttgagcagtgctttgtattttattttcttagtagcaattgtgaatgggagttcactcatgatttggctctttgtctattattggtatataggaatgcttgtgatttttgcacaccgattttgtatcctgagactttgctgaagttgcttatcagcttaaggagattttgggatgagacgatggggttttctaaatatacaatcatgtcatctgcaaacagagacaatttgacttcctctcttcctatttgaatatgctttattgctttctcttgcctgattgccctggccagaacttccaatactatgttgaataggagtggtgagagagggcatccttgccttgtgctggtcttcaaaggaaatgcttccagcttttgcccattcagtatgctattggctgtgggtttgtcataaataacctcttattatattgagatacattccatcaatacctagtttattgagggtttttagcatgaaaggctgttgaattttgttgaaggccttttttgtatctattgagataatcatgtggtttttgccgttggttctgtttatgtgatggattatgtttattgatttgcatatgttgaaccagccttgcatcccagggaagaagctgacttgatcgtggtggataagctttttgatatgctgctggattcggtttgccagtattttattgaggattttcgcatcgatgttcatcagggatattggcctaaaattctctttttttgttgtgtctctgccaggctttggtatcaggatgatgttagcctcataaaatgagttagggaggattcccttttcttctattgattggaatagtttcagaaggaatggtaccagcacctctttgtacctttcgtagaatttggctgtgaatccgtctggtcctggactttttttggttggtaggctattaattattgcctcaatttcagaacctgttactggtttattcagagattcaacttcttcctggtttagtcttgggagggtgtatgtgtcgaggaatttatccatttcttctagattttctagtttatttgtgtagaggtgtttatagtattcgctgatggtagtttgtatttctgtgggatcagtggtgatatcccctttatcattttttattgcatctatttgactcttctctcttttcttcttttttagccttgctaacggtctatcaattttgttgatcttttcaaaaaactagctcctggattcactgattttttgaagggtttgttgagtctctatctccttcagttctgctctgatcttagttatttcttgccttctgctagcttttgaatttgtttggtcttgcttctctagttcttttaattgtgatgttagggtgttgattttagatcactcctgctttcacttgtgggcatttagtgctataaatttccctctacatactgctttaaacatgtcctagagattctggtacattgtgtctttgttctcgttggttccaaagaacatctttatttctgccttcatttcgttatttacccagtagtcattcaggaacaggttgttcagtttccatgcagttgtgcagttgagtgagattcttgatcctgagttctaatttgattgcattgtggtctgagacggtttgttgtgatttctgttcttttgcatttgctgaagagtgctttacttccaattatgtggtcaattttggaataagtgtgatgtggtgctgacaagaatgtatattctgttgatttggggtggagagttctgtcgatgtctattaggtctgcttggtccagagctgagttcaagtcctggatatctttgttaattttctgtcttgttgatctgtctaatattgacagtggggtgttaaagtcacccattaatattgtgtgggagtctaaatctctttgtagaacttgctttatgaatctgggtgctcctgtattgggtgcatatatatttaggatagttagctgttcttgttgaattgatccctttaccattatgtaatgaccttctttgtctcttttgatctttgttggtttaaagtctgttttatcagagactaggattgcaacccctgcttttttctgctttccatttgcttggtaaatcttcctacatccttttattctgagcctatgtgtgtctttgcacatgagatgggtctcctgaatatagctcactgatgggtcttgactgtttattcaatttgccagtctgtgtcttttaattggggcatttatcccatttacatttaaggttaatattgttatgtgggaatttgatcctgtcattatgatgctagctggttatttcatccattaattgatgcagtttcttcatagtgttgatggtctttaccatttggcatgtttttgcagtggctggtactggttgttcctgtccattttagtgcttacttcaggagctcttgtaaggcaggcctggtggtgacaaaatctctcagcatttgcttgtctgtaaaggattttatttctccttcacttaagaagcttagtttggctggatatgagattctgggttgaaaattcttttctttaagaatgttgaatattggcccccattctcttctggcttgtagggtttctgcccagaggtccgctgttaatctgatgggcttccctttgtgggtaacctgacctttctctctggctgcccttaacagtttttccttcatttcaaccttggtgaatctgacaattatgtgtcttggggttgctcttcttgaggagtatctttgtggtgttctctgtatttcctgaatttgaatgttggccttccttgctaggttggggaagctctcctggataatatcctgaagagtgttttcaaacttggttctgttctccccatcactttcaggtacaccaatcaaacatagatttggtcttttcacatagtctcatatttcttggaggctttgttcatttcttttcactcttttttctctaatcttgtcctctcgctttatttcattaatttgatcttcagttactgatatcctttcttccacttgatcgaattggctattgaagcttgtgtatgcttcacgaagttcccgtactgtggttttcagctccatcaggtcatttaagctcttctctacactggttattctagttagccatttgtctaaccttttttcaagatttttagcttccttgcgacgcattagaacatgctcctttagcttggagaagtttgttattaccgaccttctgaagcctacttctgtcaacttgtcaaactcattctctgtccagttttgttcccttgctggcaaggagttgtgttcctttggaggagaagaggcattctggtttttggaattttcagcctttctggtctggtttctccccatctttgtggttttacctacctttggtctctgatgttggtgtcctatggatggggttttggtgtagatgtcctttttttgatgttgatgctattcctttctgttagttttccttctaatagacaggccccttagctgcaggtctgttggagtttgctggaggtccactccagaccctgtttgcctgggtgtcaccagtggaggctgcagaacagcaaatattgctgcctgatccttactgtggaagcttcgttccagtggggcatctacctctctgaggtgtctttcggcgcctactgggagatgtctcccagtcaggctacacgggggtcagggacccacttgaggaggcagtctgtctattatcggagcttgaacgcggtgctgggagaaccactgctctcttcagagctgtcaggcagggacgtttaagtctggagaagctgtctgctgccttttgttcagatatgccctgcccctggaggtggaatctacagagacagtaggccttgctgagctgtggtgggctctgcccagtttgagcttccctgctgctttgtttacactgtgagcatagaaccgcctactcaagcctcagcaatggcggacacctctaccccgccaagctcccacgtcccaggtcgatttcagactgctggcgctagcagtgagcaaggctctgtgggcgtgggacccactgaaccaggcatgggaggggatttcgtggtctgccagttgcgaagactgtgggaaaagagcagtatttgggcaggagtgtacccctcctccaggtatagtcactcacggcttcccttggctaggaaagggaaatcccccgaccccttggcgcttcccaggtgaggcgatgccccaccttgcttcggctaaccctctgtgggctacacccactgtccagccagtcccagtgagacgaaccaggtactttagttgaaaatgcagaaatcacccatcttctgtgtccatcctgctgggagctgtagactggagctgttcctattcggccatcttcaatttatttttatttttattttttgtggagacagggtctcactttgttgcccaggctggtcttgaactcctgggctcaagcagtcctcctgcctctgcctccaaagtgctagaactaaaggcatgagccaccatgcccagccctcttgaatgttttatagttttcgttatacaagtcttatacttattttgttaaatttattcctaagtatttaattctctttggtgatattgtgaacacaattttctttatttcatttttggagttttctgaacagaaaaatacaattgattttctgtatattgatctagcctgtgaccttgctgaacttgattaattctattacactatgattttttgttgtggttagacccttacacaatcaaatgaggttaaaaaaaattgtcagagtggccccagaccaacaacaggatgacagtagcctttgcccatacagagataaaatttagtttttgcagtcctttcccatagagattgtatggcagtagccaattctatggcctactgccatacaacctgaactgaagtccagaaagtttaggtgactgggccacagagctaattactggtggagccaagaagagaaattatatccctacctccttgcccactaagctccccattccagtgggctgctttctggtccttttccatgattgggctttagtagctgtcatttcctccagtgtccaagagtattttcttggccttccagtaaagctccccaagttgtctgtgttccgcctcaactgctaacttgcctacctgataaacattttgaaaagcaatctaaattctagaaattgtctctcctgcaaacaaactacagattccatttaaagcatttccttgagtccagaaagttctgagattttcctgttttggactagacttccaaagggcttcatcttaaattgtatgtatttattgacctaattgtttactgatctttagaatttagagtttaggttgggaggtcaaaatcataactttctcaatttttttggcaaactgatatgatggctggaaatcatccagaaaaagtagagatcattatattttcttgaatattcattcaagtttcaatttaatacttaaacattcattttcgaataaaaatactatgtcttgtactagggatacaaagacttggttattcttgttggagtaatgattctcctctatctggggaggtcatcctctgcagttggggactgaaggactgggagatgggagattgaaacttaaagaggtaaaggtatgtcttggaataaaactagttatcagtcaccaccagaccatcatggcggctagaattccagaaacggtgaatagaagttcatcttctattttgtcttcatggaatatatcactctggtaaacagctggttctaaatatgatggttagactttcaaggtcttcattttttagatgtaattcttcaaggagggtgtctagaaaccgtgtaaacaccataccttcctgagaatgtttctgaatgccaagaattggggtcagtaatgacagcaacaccatagcaattaaagtccattccgcaggtttgtgtataatatttctatttgttaacctgaaagttcgaacaagatttttaagttgtgtgtaaatatctcccaatgtaatctgaagaggaaccagaagcccaggcaacactttactcaacttttcaagtacgatgcgttttctaatctggttctgggaacttgagtctatcagtggaaaggtggaatcatgctcttctgagtcttgtgatttggtggtttcttcacccaaaacataccgtcctctgtaaaactccctgatcctcagatttaacttttcagtttcttttttcaaattctcgtaacttggcagtggtttaatggctgtacctgagcccctaaaaggtaaagactcatccaagctgttctgagattccctccaggcagggaaatgactatctggatctgagattatgtcatcttcatcaagttcttctttaaccagagaggcttcgggtttcagacacacagaagcataattctggccatacaaaaacctcaatgtttcttctgtcttccactcaatcaaagtctccttcaaaactttaagtaagtttctctttccaacttcaggacacacctgcactgaactagacactgacctagacacttggtttgatttggcaaattttctcttaaaatgctctgcacttttcttacttatgcctactagagttatttctgacctactgtattcactttcagaattttctgacgcttttaatctttcaggcaaagtgctatttgaagaactctgagtatttactttctgtaaaggaagttcacatgtagcatctttctcctgactatctaatttgcaatcgcctaactgctcagtgacatctactactgtctgttctttgtctttgtgtttggagttagctttgtgaccagctttctttttcattatgcttttttggtgcagctgtggtctaatatttgttgaatttggtctgtttcctggtagaatggaggaaacaaagtcttgctcattgtcactgctactatcactgtgagtgctagaagaactagattcatattgcttttcaaagtggctaggattgtcgatatctgatgttttaatggctttactgcataactgtacttcttctccagaatggccactttgttcttcctttagcagttgaaaatcaggatgcctctcttcttctcgaacccatactggagttttgggaatttgtgcttcaaaaaacttagatgcttgataacaaaaattgctgcaaaaagactttctttcagtaatatcatagactttattggttttggtagaaattttatatttctgttttggtacaattcccagcttcttctgacataaaggataaccacagagtttgacaatagaacgttcatccacgacatcactgtagtgagcaggtgtaatgaacctcccacactccattaggaactcttctgtaatattctcctctaaaagctgttcaacaatatgtagagcttttctctcaaattcaatcttctttctcacagctgcttctagttcagctttccttttagaagcatcttcttgtttcaaagtacttgtctgtttagtacctgcggcttttcgagagcagcggggagccccggccttgcggccggcagaagacggcccagcgaagtccgccatgggggagagtagtct

SEQ ID NO: 9056 - RNA, 6903 nt, Homo sapiens
  source 1..6903: mol_type = other RNA
actgagcctctctctctccagatgcccgccccactccgtgtccatagcagtgacacagccacttccccagctccgtgtaattcccaagggagcagtgaaccccaccatctcaaagctgaagagctgctggccacacacatcctctcacggttttctccctccttctgaacgccggctttgctggccctggaatctccgagtcgctctccgtgtagctgtaggcctgtgccctcgagatgcccttctgctgtcgccgccacgagttgtagtatgtggggtcactgatgtagtggttgacaaaggagtgggccttctggtggtttgagtcgacctcgtactcgctgtcacttccctgagagtcggagatttctgagggcttctccgtcaggctgctgctctctgcagggatgaggtcgttgtatttggtgacatcctcatccgagtagtgcaggctgcctgggctgggcctggggggagacctggtgtacaggccgttctttcggcagaaagagttcttgacggagagccgcctgttgttgagttccagggcagggaagctgctttcatccaagctcatcatctcgctgtggcctagggctccagacttggcactgttccccgagtctgtcttcttggcgtacttcttgctctggccccggatgatgagcacgaagaccagaagcaggatgaagatgaggccgaccagggcaatgaccaccaagaaccaccactcctcatagaaggggttggctttctgggctggcacagactgggaggggctgctgggggtgccgaaaccatagtcgttgaccgcgatgacccggaagtcatagctcacgcccggcttcaggatgtccatgctgaacgtgtaggagctcacctccttggggatgtctttgatgaggatgtcccatagtccctcgtctgaaggtctggcctcgatgacgtagcgggtgatgggccctttgcccgggtctccgctggaccagtgaatggcgatggcagagctgtaccgcacgatgatgggcacgccaggcggtcctggggcaccttctccggggcccgtggtgacgttggcttcgatctccggcccgtaggtgaaggtcttggctctgatgcggaacctgtaggtcaccccctccgccaggtccttcaccttcagccacagggggctgttccccttcacgtccacggtcacgatcttgctgactccatccacggggctgcagggctcgtacaccagcctgtagccctccaggatgccattggggaactgcggggcttcccaggacacattcactgaggttgtggtcagctcactgaacttgaccgagctgggagcgctgggggctgcttgctgggtctggccttgggtgggggtgctccgaggcccatccccagcggcgttgaaggcggccacgctgaccatgtaggccgtgtagccagtcaagttcttgagcttcacgctgttctcagccaggaaaagcgtcttcactcgctctgtgaggttcccccgctgggcttcccagaaataaatcttgtacccctggatgtctccattctggctgtccagcggaggtggctcccaagtcacgtccagctgtgtggccgtggcgccgtggacgaccacgttacgaggtgctgctgtgggcactgcctccccaacaaagacctcctgcggggggctggagggcccctcacccacagcgttgtacacgctcatccgtatctcgtaccgcctgtgcttgttcaggttgtccagctcgtactgcgtgaggctgggccggctcaggttccgcatggagtacatggaggtaagctcagcccatgtggcccctgggttgttgatgcctcgaagcgtgaagcccctcagtccttcatagagcagctcccggtatcggatccggaagcccaggaggatgccattgatcttgtcctctgctggcggctgccatcggattagcacggaggtggtggtgtggggcgtcacggagaggatggtgggtgcttcatcgggggcagcctgcagggtggtcagtgactccgactcctcgctgaactcgctgtcgccaatgtcattggtcgccttcactcggaacttgtaggacgtgaagggcttcagcctgtccacaatgaagctggaggcattgtggctcacggaggccgagtgcagtgcccacctgccgctgggcagctcgcgggtctggatggtgtagtagcgcacaggggagagcccgtcgctccctggctcccaggacagcagcacgctgcgtgctctcacatcctcctgctgcaccatcggcctgctggggggctgcggacggtctctcttctcggtggtcaccaccaaggcctcggcagcttctccccagcccttgcgggtctgggccgtgatgcggaacaggtagacagactctggcttgaggcccgtggctgtgtactgccgggcgctgggtgccagcacctccacagtggcggtgttggccgtggtggtgttgagccggtgtgtgatctggtaagcaagaatgatgccattgggggcggcagggggctgccagatcagccgcacagacgtggtccgcacctctgggaacaggatgcccatgggtggtcctgggacatcatccagcgtccgctccaggatgggagggtggctggggctgccgtccccgatgcgtgtgaaggccagcacctggacttcatagagcacgtatttgcccaagccggtgagctgggcactgcgagacgagttgccttccaccagccagaatcggggctgggtgtccgagtccttctccttatacatcaccttatagcccagcacgagcccgttgcgatcagcctcggggacctcgctccagcgcaccagcatgctgctggaggtggtggccagtgcagacacattggtggggccggaagagggaactgactcccgggtcctgcccaccaccgtctggctccagggcccgctcccgatggcgttgaaggcctggacctggacgcggtactctgtccactcctccaggtcctcgatggtgtagtcccgctccacacggtcctgcaccacgtggctcagcgtcttgccatgcccgtctgaccggctgtacttgatcttatagcccacggactcagggttcccattgtattccatctccgggagaggcatccagcgcagccacaggctggtctcactggctgtgcgcagagacacattggctggggccatgtcagggggtgcctgcagggtctggatctttctagaaggctgactgggggggctggtgcccacgatgttcacctggcgcatgcggaagctgtagcaggtgaaggggttgaggtcgggcacctccatggagcgggcatcgggctcattggagagctggtggatcagcaaccactcctctccctccccaaccacgcctacctgggcttccaccagccagcgggagatggaggttttcccatcgtagcctggcctgaactgcaaggtcacagagcgggggccgatgttggaaatgcccaggttggtggggggccctgggagttctgggggcaccccagaggagatggtggaggcggacacttggccctggccctttgaggtcatggcggccacctcgatggtgtaggtggtgagcgcggtgaggcccgtgacacggtactccagggtcacgttgggcaggtagtgggtcacacgggtgttggttcgattgtactcctcccaggagatccggtaccctgtgaggatgccatttttctctcccggctcttgccagctgaccttcagcgatgtgtccaggatctcactgaagctcaggtgtcccacgggcccaggcacatcctcatgggtgcgcaccagctgcggggtgctgcgtggcccgtccccgggggtggtgaaacacagcactgaggtgaagtactcggtgaacttcttcaggccagacacgaagcccacgtggatgctgtcttgaaagttaggccgggcggtcaccatggtaacctcctcttcctgttccggctcccaggcgatcagcttgtagccctggttgatgccgttgatgaactgggggctgggggcgttccaggtgaagcggatggtcgtggaattggtggcttccgcgtgcacattgcccggagggaccgtgggaactccctgcagcgtccactcggtgactttactgctgtagacccccagcccagcgctgttgtaagcagccacctcgatctcgtagttggtccaaatgatgagatcctccagcagcaggttgttcacatcagcatccgtgatgttcttaaactggtaccccacgggcagcccggccaggcagtacctgatgatgtaacccttgagaattccattctggtggctctcaggaggcggctgccactggatcatgatggactggttggttcgaccgctggcgatgacgttctgtggaggggccgtggggggctcctcggggagggagaccctctcggtgtctttgctgaactgtcctttccccacgtcgttgacggcacaaagacggaactggtaggagcgtgcaggaaccaggcccttgactgtcactgaggtagctttggggtccacactggccaggagtacagtccagggggcattgttctccgacatctccagaatgtagcggatcagggggctgttgccatcaaagggcttggtccacgtcaggttgatggctcgcctttccacggtgctgagagtggccactgggtgctcgggcgcgtggggcagttgcctgactcgcaggtgggcactgcgagagtcgttgcctcctgctgagatcacccggcaggtgtacgtgccgatgtctcccgaccacgtctgtgagatgtgcagggagccgtttctgtccaggcggatacgaggatggctctccgtgcccagggtggccccgtccttctcccagatgtacctgatggttactcgggggtcgtgggtcactccgcacaccatggaggcctgggtgcccttgatgacactctgatcctgggggggcttggtgatgcgggtccgagcccaaacgactaggtctgctgaggcctcatcgaccccccgagagttggtggccaggcaggtgtaggtccccgcatcggagatgtgtgtggggctgatgaggaggctgcccgactccaggggtgtgaagcgaggcagctgcacagagccactggccaagatgcgctcccctttctgccaagtgatagctggtcggggcgcccccgaggtctcacatgctagcaccactgacatgccatcgatcaccgtgctgtccagggggcctctggtgatgttaggggcgatgctggtgacagccaggtaggtggaagtttgcacctcgccggctgcattgcgggcgaagcactggaacatgccggtatcatcgggcaccaggccgctgatctgcaggcccccgtcgttgcgctgccggaagcgggtcaacttctccacctccaccacggctgcgtccttgtaccaggtgatggagggcggcggcacacctttggcctgacaggggatgtccaccaccttctccatctccgcagtgatgtgtctttctggctccttgacaaactgaggcggttccagcactgagaggtaggcgccccggacaacagaggggacgctgctgctgcgcaggacagcctcacactcgtagtagccggcgtcactgccggtggggttggggatggtgagccggcggttgtggtcactgatgccgcccgacagcaataccccgtccttcttccaaatgatatgtagcttgatcaggggcctggcattggccacacactccaaggtaacctctgaggtgccggccaccacgctggtgtttttaggtgggatgatgatggtgggtgcgatggggtctgcaggcccccctacattctccacggtgagcgtgatgggctggctggtcttgttatccccgtttttgtcgttaacagcctgcacatagtagcgacctgcgtcaggggccaccgttgacaggatgacaagggtgttctccagcgtgatggctatgcggctgctgggcgggatcttgcggccgtcccggaaccaggtcacctgtggctgggggaagctggcgatgcgcggggcacggatgacagctgcttctccgtgggagacgctctggtgcttctcaccttcctcaaagctccccatgtaggccacctggacctcggtttgccgctgcagcagggcccccattcggttccgcacgatgcaacggtaaaagccagcgtgggtgcggtccaggctggtgatcatgtatctgtattccagggagaacttggtcagctccctgttgttgtggagccacttgaactccagtggccagctgccctcggccatgcatgtaagcaccaggcggtttccttccaagtgcacctgtgtccgcacaggctctgtcttgaaatacggggacacatcatcttgggctctggccgcgcggatctgatgcagagctagcagtgtccagatcaaaagcccccacatggtgaccagcctggagaggggtcctcggggtctcccttccctccgccctgttttataatcctggtggggtccgataccccgtggcttagtcccaggaaacagtcagtctacgcggctccgtgccccggggtgtaatatgcccgggaggggcagcgcttggctaccccaacccttcctcctcttctgtactagtccgagcccggcagcgcgcccggaaggcgaggggcgagcagggagaaagaggccaggccgccctctcggactagggcgcctctctcccttagcaccccaactccgacttctcccaaacagggcggcctctgcgatccggccgggtcgccggccgagctccggaataaatggacaacttcaggaaacttcctccc

SEQ ID NO: 9057 - RNA, 7173 nt, Homo sapiens
  source 1..7173: mol_type = other RNA
actgagcctctctctctccagatgcccgccccactccgtgtccatagcagtgacacagccacttccccagctccgtgtaattcccaagggagcagtgaaccccaccatctcaaagctgaagagctgctggccacacacatcctctcacggttttctccctccttctgaacgccggctttgctggccctggaatctctggaaaaataaactcaggaggtgaaaagttgacttggtttcttggtgtttttgttttctggcaggcagtgagaggaggggtgaaggaggagtttggtgccatttctctttctgctttttcctcttctgatgtcaaacaaatgatgaaaatcctgctatgggagcccgggagcctggggccaggctgctggggggacggtagagggtgctctgctgacttggggggttaggggggttctggggcgttggagtccgactggccttgggccgaaagaggctgccctgctgggtgctggtgctgttggtgacggtggtgtggtctggctcacccgagtcgctctccgtgtagctgtaggcctgtgccctcgagatgcccttctgctgtcgccgccacgagttgtagtatgtggggtcactgatgtagtggttgacaaaggagtgggccttctggtggtttgagtcgacctcgtactcgctgtcacttccctgagagtcggagatttctgagggcttctccgtcaggctgctgctctctgcagggatgaggtcgttgtatttggtgacatcctcatccgagtagtgcaggctgcctgggctgggcctggggggagacctggtgtacaggccgttctttcggcagaaagagttcttgacggagagccgcctgttgttgagttccagggcagggaagctgctttcatccaagctcatcatctcgctgtggcctagggctccagacttggcactgttccccgagtctgtcttcttggcgtacttcttgctctggccccggatgatgagcacgaagaccagaagcaggatgaagatgaggccgaccagggcaatgaccaccaagaaccaccactcctcatagaaggggttggctttctgggctggcacagactgggaggggctgctgggggtgccgaaaccatagtcgttgaccgcgatgacccggaagtcatagctcacgcccggcttcaggatgtccatgctgaacgtgtaggagctcacctccttggggatgtctttgatgaggatgtcccatagtccctcgtctgaaggtctggcctcgatgacgtagcgggtgatgggccctttgcccgggtctccgctggaccagtgaatggcgatggcagagctgtaccgcacgatgatgggcacgccaggcggtcctggggcaccttctccggggcccgtggtgacgttggcttcgatctccggcccgtaggtgaaggtcttggctctgatgcggaacctgtaggtcaccccctccgccaggtccttcaccttcagccacagggggctgttccccttcacgtccacggtcacgatcttgctgactccatccacggggctgcagggctcgtacaccagcctgtagccctccaggatgccattggggaactgcggggcttcccaggacacattcactgaggttgtggtcagctcactgaacttgaccgagctgggagcgctgggggctgcttgctgggtctggccttgggtgggggtgctccgaggcccatccccagcggcgttgaaggcggccacgctgaccatgtaggccgtgtagccagtcaagttcttgagcttcacgctgttctcagccaggaaaagcgtcttcactcgctctgtgaggttcccccgctgggcttcccagaaataaatcttgtacccctggatgtctccattctggctgtccagcggaggtggctcccaagtcacgtccagctgtgtggccgtggcgccgtggacgaccacgttacgaggtgctgctgtgggcactgcctccccaacaaagacctcctgcggggggctggagggcccctcacccacagcgttgtacacgctcatccgtatctcgtaccgcctgtgcttgttcaggtaggtaagctcagcccatgtggcccctgggttgttgatgcctcgaagcgtgaagcccctcagtccttcatagagcagctcccggtatcggatccggaagcccaggaggatgccattgatcttgtcctctgctggcggctgccatcggattagcacggaggtggtggtgtggggcgtcacggagaggatggtgggtgcttcatcgggggcagcctgcagggtggtcagtgactccgactcctcgctgaactcgctgtcgccaatgtcattggtcgccttcactcggaacttgtaggacgtgaagggcttcagcctgtccacaatgaagctggaggcattgtggctcacggaggccgagtgcagtgcccacctgccgctgggcagctcgcgggtctggatggtgtagtagcgcacaggggagagcccgtcgctccctggctcccaggacagcagcacgctgcgtgctctcacatcctcctgctgcaccatcggcctgctggggggctgcggacggtctctcttctcggtggtcaccaccaaggcctcggcagcttctccccagcccttgcgggtctgggccgtgatgcggaacaggtagacagactctggcttgaggcccgtggctgtgtactgccgggcgctgggtgccagcacctccacagtggcggtgttggccgtggtggtgttgagccggtgtgtgatctggtaagcaagaatgatgccattgggggcggcagggggctgccagatcagccgcacagacgtggtccgcacctctgggaacaggatgcccatgggtggtcctgggacatcatccagcgtccgctccaggatgggagggtggctggggctgccgtccccgatgcgtgtgaaggccagcacctggacttcatagagcacgtatttgcccaagccggtgagctgggcactgcgagacgagttgccttccaccagccagaatcggggctgggtgtccgagtccttctccttatacatcaccttatagcccagcacgagcccgttgcgatcagcctcggggacctcgctccagcgcaccagcatgctgctggaggtggtggccagtgcagacacattggtggggccggaagagggaactgactcccgggtcctgcccaccaccgtctggctccagggcccgctcccgatggcgttgaaggcctggacctggacgcggtactctgtccactcctccaggtcctcgatggtgtagtcccgctccacacggtcctgcaccacgtggctcagcgtcttgccatgcccgtctgaccggctgtacttgatcttatagcccacggactcagggttcccattgtattccatctccgggagaggcatccagcgcagccacaggctggtctcactggctgtgcgcagagacacattggctggggccatgtcagggggtgcctgcagggtctggatctttctagaaggctgactgggggggctggtgcccacgatgttcacctggcgcatgcggaagctgtagcaggtgaaggggttgaggtcgggcacctccatggagcgggcatcgggctcattggagagctggtggatcagcaaccactcctctccctccccaaccacgcctacctgggcttccaccagccagcgggagatggaggttttcccatcgtagcctggcctgaactgcaaggtcacagagcgggggccgatgttggaaatgcccaggttggtggggggccctgggagttctgggggcaccccagaggagatggtggaggcggacacttggccctggccctttgaggtcatggcggccacctcgatggtgtaggtggtgagcgcggtgaggcccgtgacacggtactccagggtcacgttgggcaggtagtgggtcacacgggtgttggttcgattgtactcctcccaggagatccggtaccctgtgaggatgccatttttctctcccggctcttgccagctgaccttcagcgatgtgtccaggatctcactgaagctcaggtgtcccacgggcccaggcacatcctcatgggtgcgcaccagctgcggggtgctgcgtggcccgtccccgggggtggtgaaacacagcactgaggtgaagtactcggtgaacttcttcaggccagacacgaagcccacgtggatgctgtcttgaaagttaggccgggcggtcaccatggtaacctcctcttcctgttccggctcccaggcgatcagcttgtagccctggttgatgccgttgatgaactgggggctgggggcgttccaggtgaagcggatggtcgtggaattggtggcttccgcgtgcacattgcccggagggaccgtgggaactccctgcagcgtccactcggtgactttactgctgtagacccccagcccagcgctgttgtaagcagccacctcgatctcgtagttggtccaaatgatgagatcctccagcagcaggttgttcacatcagcatccgtgatgttcttaaactggtaccccacgggcagcccggccaggcagtacctgatgatgtaacccttgagaattccattctggtggctctcaggaggcggctgccactggatcatgatggactggttggttcgaccgctggcgatgacgttctgtggaggggccgtggggggctcctcggggagggagaccctctcggtgtctttgctgaactgtcctttccccacgtcgttgacggcacaaagacggaactggtaggagcgtgcaggaaccaggcccttgactgtcactgaggtagctttggggtccacactggccaggagtacagtccagggggcattgttctccgacatctccagaatgtagcggatcagggggctgttgccatcaaagggcttggtccacgtcaggttgatggctcgcctttccacggtgctgagagtggccactgggtgctcgggcgcgtggggcagttgcctgactcgcaggtgggcactgcgagagtcgttgcctcctgctgagatcacccggcaggtgtacgtgccgatgtctcccgaccacgtctgtgagatgtgcagggagccgtttctgtccaggcggatacgaggatggctctccgtgcccagggtggccccgtccttctcccagatgtacctgatggttactcgggggtcgtgggtcactccgcacaccatggaggcctgggtgcccttgatgacactctgatcctgggggggcttggtgatgcgggtccgagcccaaacgactaggtctgctgaggcctcatcgaccccccgagagttggtggccaggcaggtgtaggtccccgcatcggagatgtgtgtggggctgatgaggaggctgcccgactccaggggtgtgaagcgaggcagctgcacagagccactggccaagatgcgctcccctttctgccaagtgatagctggtcggggcgcccccgaggtctcacatgctagcaccactgacatgccatcgatcaccgtgctgtccagggggcctctggtgatgttaggggcgatgctggtgacagccaggtaggtggaagtttgcacctcgccggctgcattgcgggcgaagcactggaacatgccggtatcatcgggcaccaggccgctgatctgcaggcccccgtcgttgcgctgccggaagcgggtcaacttctccacctccaccacggctgcgtccttgtaccaggtgatggagggcggcggcacacctttggcctgacaggggatgtccaccaccttctccatctccgcagtgatgtgtctttctggctccttgacaaactgaggcggttccagcactgagaggtaggcgccccggacaacagaggggacgctgctgctgcgcaggacagcctcacactcgtagtagccggcgtcactgccggtggggttggggatggtgagccggcggttgtggtcactgatgccgcccgacagcaataccccgtccttcttccaaatgatatgtagcttgatcaggggcctggcattggccacacactccaaggtaacctctgaggtgccggccaccacgctggtgtttttaggtgggatgatgatggtgggtgcgatggggtctgcaggcccccctacattctccacggtgagcgtgatgggctggctggtcttgttatccccgtttttgtcgttaacagcctgcacatagtagcgacctgcgtcaggggccaccgttgacaggatgacaagggtgttctccagcgtgatggctatgcggctgctgggcgggatcttgcggccgtcccggaaccaggtcacctgtggctgggggaagctggcgatgcgcggggcacggatgacagctgcttctccgtgggagacgctctggtgcttctcaccttcctcaaagctccccatgtaggccacctggacctcggtttgccgctgcagcagggcccccattcggttccgcacgatgcaacggtaaaagccagcgtgggtgcggtccaggctggtgatcatgtatctgtattccagggagaacttggtcagctccctgttgttgtggagccacttgaactccagtggccagctgccctcggccatgcatgtaagcaccaggcggtttccttccaagtgcacctgtgtccgcacaggctctgtcttgaaatacggggacacatcatcttgggctctggccgcgcggatctgatgcagagctagcagtgtccagatcaaaagcccccacatggtgaccagcctggagaggggtcctcggggtctcccttccctccgccctgttttataatcctggtggggtccgataccccgtggcttagtcccaggaaacagtcagtctacgcggctccgtgccccggggtgtaatatgcccgggaggggcagcgcttggctaccccaacccttcctcctcttctgtactagtccgagcccggcagcgcgcccggaaggcgaggggcgagcagggagaaagaggccaggccgccctctcggactagggcgcctctctcccttagcaccccaactccgacttctcccaaacagggcggcctctgcgatccggccgggtcgccggccgagctccggaataaatggacaacttcaggaaacttcctc

SEQ ID NO: 9058 - RNA, 7203 nt, Homo sapiens
  source 1..7203: mol_type = other RNA
actgagcctctctctctccagatgcccgccccactccgtgtccatagcagtgacacagccacttccccagctccgtgtaattcccaagggagcagtgaaccccaccatctcaaagctgaagagctgctggccacacacatcctctcacggttttctccctccttctgaacgccggctttgctggccctggaatctctggaaaaataaactcaggaggtgaaaagttgacttggtttcttggtgtttttgttttctggcaggcagtgagaggaggggtgaaggaggagtttggtgccatttctctttctgctttttcctcttctgatgtcaaacaaatgatgaaaatcctgctatgggagcccgggagcctggggccaggctgctggggggacggtagagggtgctctgctgacttggggggttaggggggttctggggcgttggagtccgactggccttgggccgaaagaggctgccctgctgggtgctggtgctgttggtgacggtggtgtggtctggctcacccgagtcgctctccgtgtagctgtaggcctgtgccctcgagatgcccttctgctgtcgccgccacgagttgtagtatgtggggtcactgatgtagtggttgacaaaggagtgggccttctggtggtttgagtcgacctcgtactcgctgtcacttccctgagagtcggagatttctgagggcttctccgtcaggctgctgctctctgcagggatgaggtcgttgtatttggtgacatcctcatccgagtagtgcaggctgcctgggctgggcctggggggagacctggtgtacaggccgttctttcggcagaaagagttcttgacggagagccgcctgttgttgagttccagggcagggaagctgctttcatccaagctcatcatctcgctgtggcctagggctccagacttggcactgttccccgagtctgtcttcttggcgtacttcttgctctggccccggatgatgagcacgaagaccagaagcaggatgaagatgaggccgaccagggcaatgaccaccaagaaccaccactcctcatagaaggggttggctttctgggctggcacagactgggaggggctgctgggggtgccgaaaccatagtcgttgaccgcgatgacccggaagtcatagctcacgcccggcttcaggatgtccatgctgaacgtgtaggagctcacctccttggggatgtctttgatgaggatgtcccatagtccctcgtctgaaggtctggcctcgatgacgtagcgggtgatgggccctttgcccgggtctccgctggaccagtgaatggcgatggcagagctgtaccgcacgatgatgggcacgccaggcggtcctggggcaccttctccggggcccgtggtgacgttggcttcgatctccggcccgtaggtgaaggtcttggctctgatgcggaacctgtaggtcaccccctccgccaggtccttcaccttcagccacagggggctgttccccttcacgtccacggtcacgatcttgctgactccatccacggggctgcagggctcgtacaccagcctgtagccctccaggatgccattggggaactgcggggcttcccaggacacattcactgaggttgtggtcagctcactgaacttgaccgagctgggagcgctgggggctgcttgctgggtctggccttgggtgggggtgctccgaggcccatccccagcggcgttgaaggcggccacgctgaccatgtaggccgtgtagccagtcaagttcttgagcttcacgctgttctcagccaggaaaagcgtcttcactcgctctgtgaggttcccccgctgggcttcccagaaataaatcttgtacccctggatgtctccattctggctgtccagcggaggtggctcccaagtcacgtccagctgtgtggccgtggcgccgtggacgaccacgttacgaggtgctgctgtgggcactgcctccccaacaaagacctcctgcggggggctggagggcccctcacccacagcgttgtacacgctcatccgtatctcgtaccgcctgtgcttgttcaggttgtccagctcgtactgcgtgaggctgggccggctcaggttccgcatggagtacatggaggtaagctcagcccatgtggcccctgggttgttgatgcctcgaagcgtgaagcccctcagtccttcatagagcagctcccggtatcggatccggaagcccaggaggatgccattgatcttgtcctctgctggcggctgccatcggattagcacggaggtggtggtgtggggcgtcacggagaggatggtgggtgcttcatcgggggcagcctgcagggtggtcagtgactccgactcctcgctgaactcgctgtcgccaatgtcattggtcgccttcactcggaacttgtaggacgtgaagggcttcagcctgtccacaatgaagctggaggcattgtggctcacggaggccgagtgcagtgcccacctgccgctgggcagctcgcgggtctggatggtgtagtagcgcacaggggagagcccgtcgctccctggctcccaggacagcagcacgctgcgtgctctcacatcctcctgctgcaccatcggcctgctggggggctgcggacggtctctcttctcggtggtcaccaccaaggcctcggcagcttctccccagcccttgcgggtctgggccgtgatgcggaacaggtagacagactctggcttgaggcccgtggctgtgtactgccgggcgctgggtgccagcacctccacagtggcggtgttggccgtggtggtgttgagccggtgtgtgatctggtaagcaagaatgatgccattgggggcggcagggggctgccagatcagccgcacagacgtggtccgcacctctgggaacaggatgcccatgggtggtcctgggacatcatccagcgtccgctccaggatgggagggtggctggggctgccgtccccgatgcgtgtgaaggccagcacctggacttcatagagcacgtatttgcccaagccggtgagctgggcactgcgagacgagttgccttccaccagccagaatcggggctgggtgtccgagtccttctccttatacatcaccttatagcccagcacgagcccgttgcgatcagcctcggggacctcgctccagcgcaccagcatgctgctggaggtggtggccagtgcagacacattggtggggccggaagagggaactgactcccgggtcctgcccaccaccgtctggctccagggcccgctcccgatggcgttgaaggcctggacctggacgcggtactctgtccactcctccaggtcctcgatggtgtagtcccgctccacacggtcctgcaccacgtggctcagcgtcttgccatgcccgtctgaccggctgtacttgatcttatagcccacggactcagggttcccattgtattccatctccgggagaggcatccagcgcagccacaggctggtctcactggctgtgcgcagagacacattggctggggccatgtcagggggtgcctgcagggtctggatctttctagaaggctgactgggggggctggtgcccacgatgttcacctggcgcatgcggaagctgtagcaggtgaaggggttgaggtcgggcacctccatggagcgggcatcgggctcattggagagctggtggatcagcaaccactcctctccctccccaaccacgcctacctgggcttccaccagccagcgggagatggaggttttcccatcgtagcctggcctgaactgcaaggtcacagagcgggggccgatgttggaaatgcccaggttggtggggggccctgggagttctgggggcaccccagaggagatggtggaggcggacacttggccctggccctttgaggtcatggcggccacctcgatggtgtaggtggtgagcgcggtgaggcccgtgacacggtactccagggtcacgttgggcaggtagtgggtcacacgggtgttggttcgattgtactcctcccaggagatccggtaccctgtgaggatgccatttttctctcccggctcttgccagctgaccttcagcgatgtgtccaggatctcactgaagctcaggtgtcccacgggcccaggcacatcctcatgggtgcgcaccagctgcggggtgctgcgtggcccgtccccgggggtggtgaaacacagcactgaggtgaagtactcggtgaacttcttcaggccagacacgaagcccacgtggatgctgtcttgaaagttaggccgggcggtcaccatggtaacctcctcttcctgttccggctcccaggcgatcagcttgtagccctggttgatgccgttgatgaactgggggctgggggcgttccaggtgaagcggatggtcgtggaattggtggcttccgcgtgcacattgcccggagggaccgtgggaactccctgcagcgtccactcggtgactttactgctgtagacccccagcccagcgctgttgtaagcagccacctcgatctcgtagttggtccaaatgatgagatcctccagcagcaggttgttcacatcagcatccgtgatgttcttaaactggtaccccacgggcagcccggccaggcagtacctgatgatgtaacccttgagaattccattctggtggctctcaggaggcggctgccactggatcatgatggactggttggttcgaccgctggcgatgacgttctgtggaggggccgtggggggctcctcggggagggagaccctctcggtgtctttgctgaactgtcctttccccacgtcgttgacggcacaaagacggaactggtaggagcgtgcaggaaccaggcccttgactgtcactgaggtagctttggggtccacactggccaggagtacagtccagggggcattgttctccgacatctccagaatgtagcggatcagggggctgttgccatcaaagggcttggtccacgtcaggttgatggctcgcctttccacggtgctgagagtggccactgggtgctcgggcgcgtggggcagttgcctgactcgcaggtgggcactgcgagagtcgttgcctcctgctgagatcacccggcaggtgtacgtgccgatgtctcccgaccacgtctgtgagatgtgcagggagccgtttctgtccaggcggatacgaggatggctctccgtgcccagggtggccccgtccttctcccagatgtacctgatggttactcgggggtcgtgggtcactccgcacaccatggaggcctgggtgcccttgatgacactctgatcctgggggggcttggtgatgcgggtccgagcccaaacgactaggtctgctgaggcctcatcgaccccccgagagttggtggccaggcaggtgtaggtccccgcatcggagatgtgtgtggggctgatgaggaggctgcccgactccaggggtgtgaagcgaggcagctgcacagagccactggccaagatgcgctcccctttctgccaagtgatagctggtcggggcgcccccgaggtctcacatgctagcaccactgacatgccatcgatcaccgtgctgtccagggggcctctggtgatgttaggggcgatgctggtgacagccaggtaggtggaagtttgcacctcgccggctgcattgcgggcgaagcactggaacatgccggtatcatcgggcaccaggccgctgatctgcaggcccccgtcgttgcgctgccggaagcgggtcaacttctccacctccaccacggctgcgtccttgtaccaggtgatggagggcggcggcacacctttggcctgacaggggatgtccaccaccttctccatctccgcagtgatgtgtctttctggctccttgacaaactgaggcggttccagcactgagaggtaggcgccccggacaacagaggggacgctgctgctgcgcaggacagcctcacactcgtagtagccggcgtcactgccggtggggttggggatggtgagccggcggttgtggtcactgatgccgcccgacagcaataccccgtccttcttccaaatgatatgtagcttgatcaggggcctggcattggccacacactccaaggtaacctctgaggtgccggccaccacgctggtgtttttaggtgggatgatgatggtgggtgcgatggggtctgcaggcccccctacattctccacggtgagcgtgatgggctggctggtcttgttatccccgtttttgtcgttaacagcctgcacatagtagcgacctgcgtcaggggccaccgttgacaggatgacaagggtgttctccagcgtgatggctatgcggctgctgggcgggatcttgcggccgtcccggaaccaggtcacctgtggctgggggaagctggcgatgcgcggggcacggatgacagctgcttctccgtgggagacgctctggtgcttctcaccttcctcaaagctccccatgtaggccacctggacctcggtttgccgctgcagcagggcccccattcggttccgcacgatgcaacggtaaaagccagcgtgggtgcggtccaggctggtgatcatgtatctgtattccagggagaacttggtcagctccctgttgttgtggagccacttgaactccagtggccagctgccctcggccatgcatgtaagcaccaggcggtttccttccaagtgcacctgtgtccgcacaggctctgtcttgaaatacggggacacatcatcttgggctctggccgcgcggatctgatgcagagctagcagtgtccagatcaaaagcccccacatggtgaccagcctggagaggggtcctcggggtctcccttccctccgccctgttttataatcctggtggggtccgataccccgtggcttagtcccaggaaacagtcagtctacgcggctccgtgccccggggtgtaatatgcccgggaggggcagcgcttggctaccccaacccttcctcctcttctgtactagtccgagcccggcagcgcgcccggaaggcgaggggcgagcagggagaaagaggccaggccgccctctcggactagggcgcctctctcccttagcaccccaactccgacttctcccaaacagggcggcctctgcgatccggccgggtcgccggccgagctccggaat

SEQ ID NO: 9059 - RNA, 1348 nt, Homo sapiens
  source 1..1348: mol_type = other RNA
actgagcctctctctctccaggtgaagtttgtgcaagcgtgagttaagagatttgatgaaattattcacccagatgtaagtgtcggtatgttattaatactttctccaagaacatgcacatcttcacctgggcttgctgctgccccacgtagtaaggatgcaacagtttgtggttctctagagagctttgccaccagttttgcagggagagggcttttagtgtcttagccatagtgacatgtaaacaattgatatgagagtttttcttgagaatgaatttttatacaaagaaaagggagaggaagagaacattgctggccttggaaatctcaaataaaaggctacgcatgggctcaatatatcatctcaatgaaatggaggtgacagaggatggaatccgtgaccttgaggatagctcagtggaatttgttccatcttatacagcggacgccgcacatcgatggggcagttctgtattacttcatcaacaacatctgagatggactccatagagtctgggttggcaaactccgggtgaaagaatatttcaggtcccaggaatctttcgtaaccaacgtctataacaaacttcttctggttgatcgcattgatacccgtgtactgtttgatccacttctggggatccacatcatacttggcaaattccttgactatatcggggcaaatgtaacagtatttctccttaatggcttttgcggtctccagtgactgctcaggagggattcccacctccctctcccttagcagctgttgaatgaaatacgtaatatctctacctgcaatcgggatgtgtttgatgcagcttccaattacataaccttctgccactgggataacatgggtgactccatctccgctgtcaatgactatccccgttaatgtacgttcacccacttgtcgagatgtccaagatgccgccaaggccagcactgcctgaactgcaatgtagagtcctggaacgttaaatgattcgaacataatttctgcaagatactctctgttttctggtgtattgagtggaggttctgtcgatagatgagccttccacgcgggagacctggatccttatcgtctttgtggccccttccatctgcacgtgcggacgaggtccgggtcgcactcgggcggtcagcctggcacgcacagcgccggcgtgcagggggccttgggtgccaccgagtccgggaggaaatctaggccgccatccgtccggagactggcacctgtgaccaccacccaacatgtattgaacaagggcttggaggtcctttctctaaggccgcaccgataaacgattaccgactgttgacctcacggccccttcgct

SEQ ID NO: 9060 - RNA, 1127 nt, Homo sapiens
  source 1..1127: mol_type = other RNA
actgagcctctctctctccaggtgaagtttgtgcaagcgtgagttaagagatttgatgaaattattcacccagatgtaagtgtcggtatgttattaatactttctccaagaacatgcacatcttcacctgggcttgctgctgccccacgtagtaaggatgcaacagtttgtggttctctagagagctttgccaccagttttgcagggagagggcttttagtgtcttagccatagtgacatgtaaacaattgatatgagagtttttcttgagaatgaatttttatacaaagaaaagggagaggaagagaacattgctggccttggaaatctcaaataaaaggctacgcatgggctcaatatatcatctcaatgaaatggaggtgacagaggatggaatccgtgaccttgaggatagctcagtggaatttgttccatcttatacagcggacgccgcacatcgatggggcagttctgtattacttcatcaacaacatctgagatggactccatagagtctgggttggcaaactccgggtgaaagaatatttcaggtcccaggaatctttcgtaaccaacgtctataacaaacttcttctggttgatcgcattgatacccgtgtactgtttgatccacttctggggatccacatcatacttggcaaattccttgactatatcggggcaaatgtaacagtatttctccttaatggcttttgcggtctccagtgactgctcaggagggattcccacctccctctcccttagcagctgttgaatgaaatacgtaatatctctacctgcaatcgggatgtgtttgatgcagcttccaattacataaccttctgccactgggataacatgggtgactccatctccgctgtcaatgactatccccgttaatgtacgttcacccacttgtcgagatgtccaagatgccgccaaggccagcactgcctgaactgcaatgtagagtcctggaacgttaaatgattcgaacataatttctgcaagatactctctgttttctggtgtattgagtggaggttctgtctgccgaggaggcgccggctctgcggtgcggagttgcgccggacttcccagcttggccagtggctccgcaggctgcc

SEQ ID NO: 9061 - RNA, 1272 nt, Homo sapiens
  source 1..1272: mol_type = other RNA
actgagcctctctctctccaggtgaagtttgtgcaagcgtgagttaagagatttgatgaaattattcacccagatgtaagtgtcggtatgttattaatactttctccaagaacatgcacatcttcacctgggcttgctgctgccccacgtagtaaggatgcaacagtttgtggttctctagagagctttgccaccagttttgcagggagagggcttttagtgtcttagccatagtgacatgtaaacaattgatatgagagtttttcttgagaatgaatttttatacaaagaaaagggagaggaagagaacattgctggccttggaaatctcaaataaaaggctacgcatgggctcaatatatcatctcaatgaaatggaggtgacagaggatggaatccgtgaccttgaggatagctcagtggaatttgttccatcttatacagcggacgccgcacatcgatggggcagttctgtattacttcatcaacaacatctgagatggactccatagagtctgggttggcaaactccgggtgaaagaatatttcaggtcccaggaatctttcgtaaccaacgtctataacaaacttcttctggttgatcgcattgatacccgtgtactgtttgatccacttctggggatccacatcatacttggcaaattccttgactatatcggggcaaatgtaacagtatttctccttaatggcttttgcggtctccagtgactgctcaggagggattcccacctccctctcccttagcagctgttgaatgaaatacgtaatatctctacctgcaatcgggatgtgtttgatgcagcttccaattacataaccttctgccactgggataacatgggtgactccatctccgctgtcaatgactatccccgttaatgtacgttcacccacttgtcgagatgtccaagatgccgccaaggccagcactgcctgaactgcaatgtagagtcctggaacgttaaatgattcgaacataatttctgcaagatactctctgttttctggtgtattgagtggaggttctgtggcagcaagatggcaatgccaagcaggagacgcagcacatcttgccacagcttcctcctggccagaggctccctaacatgggtgacactctccacataggtaaaatccagccagagttgtgaaagcagctgaatctctcccttgctactgtcttcatgcctttgagtgacaccactatgacaggcattgagttgctcttaccaacactgcaagtttgtgact

SEQ ID NO: 9062 - RNA, 2343 nt, Homo sapiens
  source 1..2343: mol_type = other RNA
actgagcctctctctctccaggtgaagtttgtgcaagcgtgagttaagagatttgatgaaattattcacccagatgtaagtgtcggtatgttattaatactttctccaagaacatgcacatcttcacctgggcttgctgctgccccacgtagtaaggatgcaacagtttgtggttctctagagagctttgccaccagttttgcagggagagggcttttagtgtcttagccatagtgacatgtaaacaattgatatgagagtttttcttgagaatgaatttttatacaaagaaaagggagaggaagagaacattgctggccttggaaatctgaaaaacagacacaaaacaggaaaggaaagaaagcagattatttagtttaccgtcttcataatttaaggttaatgtagttttgatatgcccccaccaaatctcgtgttgaactgtaatctccactcttggaggcggggcctggtgggggtgtttatatcatgggagtgcattcctcatggatggcgtgggccatctcttgggtgatgagtgagctctgagttcacaagagatctggtcatgtagaagtgtgtggcaactgcctcccactcttttgttcttgcttttgccatgtgaagtgcctgctcccacttcaccttcctctgtgagtcaaagctccctgagccctccccagaagctgggcaccatgctggtacagccttcaggcttgtgagccaattgaacctcttttctttaaaaattaccccatctcaggatctggggcaaaggtactccaacaatagacgatgctgttggcaatacctgctcgattccagccaaactacaatggaacctgcccctgccagggtttcagcagggccaagctggaagctgattttccaccctagctcctgtcccagggaagcaggccatgggctccagtttctctgcggtgtcagcaggatgcagagtaagcccacttccaccaggcatcgatgatacagaatgaggcaactcaaggtagagtggtccgcgttctgctctcccttccctcccgtactggccctgggcccaaaggagactgaacagatacacagccctggtgctacatctcaacagagaagctggctattaaaaaaaaaaaagagtaggccgggtgcggtggctcgcacctgtaatcccaacactttgggaggccgaggtgggcagatcacgagatcaggagatcgagaacatcctggccaacatggtgaaaccccatctctactaaaaatacaaaaatgagctgggtgtggtggcgcatgtttgcaatcccagctactcaggaggctgtggcaggagaatcgattgaacccaggaggcagaggttgcagtgagctgagatcgcaccactgcactccagcctggagatagagctagactccgtctcaaaaaaaaaaaaagtaaataggattcacaatcttatcaaaatgtccagaatacaataaaaaaccacttatcatagcaagaaccagaaaaatcacaaatgaatgaagagtcgattgagactccaacataaagatgactcaggtgctgggattacctgcaaagaattttagaataattgtcataaaaatgcttcaataagcaattatgggttctcttgaaacaaatgaaaaaaatagaaaatttcagcaaaagtagagcctagaattaaaaatgaaaatcatgagaatacctcaaataaaaggctacgcatgggctcaatatatcatctcaatgaaatggaggtgacagaggatggaatccgtgaccttgaggatagctcagtggaatttgttccatcttatacagcggacgccgcacatcgatggggcagttctgtattacttcatcaacaacatctgagatggactccatagagtctgggttggcaaactccgggtgaaagaatatttcaggtcccaggaatctttcgtaaccaacgtctataacaaacttcttctggttgatcgcattgatacccgtgtactgtttgatccacttctggggatccacatcatacttggcaaattccttgactatatcggggcaaatgtaacagtatttctccttaatggcttttgcggtctccagtgactgctcaggagggattcccacctccctctcccttagcagctgttgaatgaaatacgtaatatctctacctgcaatcgggatgtgtttgatgcagcttccaattacataaccttctgcaagatactctctgttttctggtgtattgagtggaggttctgtctgccgaggaggcgccggctctgcggtgcggagttgcgccggacttcccagcttggccagtggctccgcaggctgcc

SEQ ID NO: 9063 - RNA, 213 nt, Homo sapiens
  source 1..213: mol_type = other RNA
actgccctaagtgctccttctggggacctgaggagggcataggcagcatggcccacgtacccacctctcaagagaggcctccagcaatgcctccttttagccacaggtcctgggaccagtgagccagggcctacagcagcccacatggacacatggacacatggaaacgtggccacactgccacagagtcaagagcccttctccctgctgagc

SEQ ID NO: 9064 - RNA, 2520 nt, Homo sapiens
  source 1..2520: mol_type = other RNA
actggactaggagtcagaaggcctatattccagtctcaattctgctgttaactcagtgtgcggccttgggggcaagtcccttcctacctccaggcctcagttttcccatctgtaaaataagggcattgaactagattaatagttaagattccttccagctctaacgttttatgactttttatgtccattattaacgcctgagccatgcagtctcagggaagttagcttctaagagagaacatacctctgtatcctttgctttgttcatttagctataaagcacgtctgcctttggcacttgggtcagacatacaaagttatgagcatcctgatttactatcctactcagcatgctagtggaatctgtcagcactataagttgattattgagaaagggagaaaaactccaactagttaaacctggaaatataagataacttcgcctcatgcgctcacgaacaggtgagagtggttgtgagcacacacacacatcgggatacacactattgctagtgatcagttcattacagtaatccatttcccttaataaaaattagtaaatagtatagcatagcaaagtttggcatctaaggaaacatctatggaaaaacagcacttttggacatgttagagaaaaagggacaggtagagagagacaaatatagatcaaatgagatagaaatacaggcagagaaaggatcagtctgaaaaagaaggaggggagaaggagaaagggaggaagaaagagaaaaagtaaaagcagacagggtgagaatgaaggggaaaggaatacagaacagaataatgaaagaggagagaggaataaagaagagaagggcagtaacagggagaaggggtcgtattccctggaaggttgaacgctgttccacatgtacctgtgaaaaccatcttagaagaaagcttccaaaggcacagcagaaaacagagtgacgatcagagcctgcatcgagaggtattacattggggagcccctaaacctccacgttgctggccctgtcagtcctcagtgttcaaacctcatacccatatatcacctgaatttgccatgacaaccataaaggctgagctggcagggtgtaaagactgaagaggagtgggatagatactgtgagaaagaacaaggcatcctgcaccaggatgtacttggtcattcccctgacactgcaggaacaaaagagaggccctaactttggctagtttatcactcctccccctctccaaagatgaggcctatgctttgctgttggggactcgaaggagaaaagctctggatccaccttgttggaaggtcatacagacttttcctgggccttggggaagggtgcactaccagaagagatctttctgcacacagtgttggtgtgcctcttgcagcggcagcctggtcgccggaggctatcatagccctgttggcacagatggaggcatccacgggtaggcaggtagcagcacaggcagggtaggaagagggagatgaggctcatggctgcccagcggacaaagcaagaactaggcccacaagagcagggctcatcagcacagttgtcttcatcatcagtggagcagtggtagaagaggcccttgacacagcagagacaagtgccataatcgaggaggctctcagcagagcaaaggcagcgctggttgcacagccagcaggaggggagagggcgagctgctgtgcaggggacgcacttgcagcgcccacattcctcacagatgaagaggtgctcactagggtgccctgcagattgctcagcttctcccttcagagcaccatcagcctttgggtggacccctgctccaggttgggttcggatgatggattggcctgaaggtgagggtgtaatgctggccaagagcctttgatcagaggcagtggtgctatgggacattgagctggcaatgctagattggctcagatgctgaggcaagggctgcagttgatggcactggctgagactgcgggggagagaagtaggcatggtagccagagaccaatcagacttgtgggtttgcacaataagggaagggctggagagggcctgtttacagggggctggaggccgttccacgtagtcattgctagcatgagtagagcgcagctgttcaataggcagaatttgttgaaaatcatctgtcaccgcagcatccattttgccttgattttttagctctgagtggttttaagtcagggtggcacttatggtgataaagaggagcccttgtagttacatggatttcagggcacatgagaaaatccttgaggaaatggtttatccatgctgagaaaagcagaagaactaatgccccatctggctcaaaggatctcttctcctcagtctttaggtttctccacctctcttcggaaagtctgaatgaaaactccttcactggcaggcagtggagccagaaacagagatagttctgtcttgttcttaaccctggcggagaggaaggccactcctgccttgccgcagggttgtcgtcacgatctgt

SEQ ID NO: 9065 - RNA, 2685 nt, Homo sapiens
  source 1..2685: mol_type = other RNA
actggactaggagtcagaaggcctatattccagtctcaattctgctgttaactcagtgtgcggccttgggggcaagtcccttcctacctccaggcctcagttttcccatctgtaaaataagggcattgaactagattaatagttaagattccttccagctctaacgttttatgactttttatgtccattattaacgcctgagccatgcagtctcagggaagttagcttctaagagagaacatacctctgtatcctttgctttgttcatttagctataaagcacgtctgcctttggcacttgggtcagacatacaaagttatgagcatcctgatttactatcctactcagcatgctagtggaatctgtcagcactataagttgattattgagaaagggagaaaaactccaactagttaaacctggaaatataagataacttcgcctcatgcgctcacgaacaggtgagagtggttgtgagcacacacacacatcgggatacacactattgctagtgatcagttcattacagtaatccatttcccttaataaaaattagtaaatagtatagcatagcaaagtttggcatctaaggaaacatctatggaaaaacagcacttttggacatgttagagaaaaagggacaggtagagagagacaaatatagatcaaatgagatagaaatacaggcagagaaaggatcagtctgaaaaagaaggaggggagaaggagaaagggaggaagaaagagaaaaagtaaaagcagacagggtgagaatgaaggggaaaggaatacagaacagaataatgaaagaggagagaggaataaagaagagaagggcagtaacagggagaaggggtcgtattccctggaaggttgaacgctgttccacatgtacctgtgaaaaccatcttagaagaaagcttccaaaggcacagcagaaaacagagtgacgatcagagcctgcatcgagaggtattacattggggagcccctaaacctccacgttgctggccctgtcagtcctcagtgttcaaacctcatacccatatatcacctgaatttgccatgacaaccataaaggctgagctggcagggtgtaaagactgaagaggagtgggatagatactgtgagaaagaacaaggcatcctgcaccaggatgtacttggtcattcccctgacactgcaggaacaaaagagaggccctaactttggctagtttatcactcctccccctctccaaagatgaggcctatgctttgctgttggggactcgaaggagaaaagctctggatccaccttgttggaaggtcatacagacttttcctgggccttggggaagggtgcactaccagaagagatctttctgcacacagtgttggtgtgcctcttgcagcggcagcctggtcgccggaggctatcatagccctgttggcacagatggaggcatccacgggtaggcaggtagcagcacaggcagggtaggaagagggagatgaggctcatggctgcccagcggacaaagcaagaactaggcccacaagagcagggctcatcagcacagttgtcttcatcatcagtggagcagtggtagaagaggcccttgacacagcagagacaagtgccataatcgaggaggctctcagcagagcaaaggcagcgctggttgcacagccagcaggaggggagagggcgagctgctgtgcaggggacgcacttgcagcgcccacattcctcacagatgaagaggtgctcactagggtgccctgcagattgctcagcttctcccttcagagcaccatcagcctttgggtggacccctgctccaggttgggttcggatgatggattggcctgaaggtgagggtgtaatgctggccaagagcctttgatcagaggcagtggtgctatgggacattgagctggcaatgctagattggctcagatgctgaggcaagggctgcagttgatggcactggctgagactgcgggggagagaagtaggcatggtagccagagaccaatcagacttgtgggtttgcacaataagggaagggctggagagggcctgtttacagggggctggaggccgttccacgtagtcattgctagcatgagtagagcgcagctgttcaataggcagaatttgttgaaaatcatctgtcaccgcagcatccattttgccttgattttttagctctgagtggttttaagtcagggtggcacttatggtgataaagaggagcccttgtagttacatggatttcagggcacatgagaaaatccttgaggaaatggtttatccatgctgagaaaagcagaagaactaatgccccatctggctcaaaggatctcttctcctcagtctttaggtttctccacctctcttcggaaagtctgaatgaaaactccttcactggcaggcagtggagccagaaacagagatagttctgtcttgttctttgacacagcagagaaaacacaaaacaaaacaaaacaaaacaaaacaaaacaaaaaaacgggggagggggcgagtcaaacctgtagtggcatatactttgtatagattttacaggcagatctaaatcttgatggacgtatttcccaaagaaagctcagcagggtaagttgttcacctcctcctctttctcctcctcctcctctctctcctcctcctcctctctct

SEQ ID NO: 9066 - RNA, 4286 nt, Homo sapiens
  source 1..4286: mol_type = other RNA
actggacttggagtcagaaagacctaggttcgaatcagcactctgtcacatgtggccctgaacaagcttctcaagcatcacgactcagtttcatgcataaaatgatgagtgatggtacctacctcccttgctaaacatttaaagaggccacacacgaatagcactttacaaagaacccagctaagaatcagcactcaataaaggacagataccatcagggctcaggagccagccctctggggacctcccccaaggagcaggaagaaccaacccactaagcagcaagagtctagccagaatttcctcatctcctcaggaaaagaaaaaaaaaaactcagatctcgatgcttcctctttaaggatcatttttaactgcaggttctggccagggacctccacttcaattcaaaaggagcaccctgaagaaatggcagaagttgagatgggaacacgaccaggccaagcagggcagcccctcagtgatccaagaccaccacctgcagcaaacactgcaaggccagaaatctgctctgctcttttctccagcaatgggatcaattacaccctcagaggggctggtctgggggctaaatgccagtcctcacctgctccacactattgctgccatagctcagcaagagacagccaagaccccaaggcagagggacaagtccatccctgcttgaaacaacagcctggaggaaaagcagcccattctgcctcctgagggcgatcccctagctggtgggcacactgtgcatcctcccatgcaggaaagagcacagggctatgggtccttctcctcgtttcttgggggacaaagcactcaggaccccatcccttgggcctccagggaaagcaaggctccagaggcacagttgtctgaatgggtaacaggaaagagttcttggatcactaactgctctgccagtggagtttaaccccaaaacattcactggttccagcacaagtttcaaaatcaaaccactgagtgcccaaataattaaatggatcacgttatctcacctcacccttgccatcgcacagaagggggctacgcccattgtgagcaactgttctttggcaggggaagagagacaaaggtaggagggaaatgaattacaaaagggaaaacaagcctatttggagatttcaagcaagactgggtcctaaggattagttcactaacctactcagaaggctgacactgcctgctacctagagtctgcaataatgccttgaaatgttattagcagggcttccccctcccagaggccacagcctttactgggcccaggtccttcctttcaagtctctctcatcacaaaggccctctcaccccttcaattccaaaggcactggatatccctcagcctctcagcccctcaacctctcgatgtgccttcaggtactctgctttccccttgctaacccttagctaactcaccctttctacctctgctgacatagaattccctccctccccacaaaaacctgccctcccccaaaaacaaattttgtcccctactgtacacgaaaccctgtacttctccttggcagcaccttgccaggtttgcttaaagggcttccttcttgatggactgtaagctccatgaaggcagggaccactctgagattacctactataaccctagcccaaatatttcaataccccaacaataccccaacctgactttccaacttcacctccctccccaagtacttcagcctccagccatacccctcaaggttccaaaatcgccatgcttttactaccactgctctataaaaaacccaggtcacctctcaaggctctgctaaaggccaactgccccaggaaatctttcccaatctcccagcaatacacatgcctctcaccttcaccctggtggaaataatcaagcaagagagccacaaggacctaccttctaatcagattcccactaactaggggagtgagcttggacaagtcattaagctggagcctcattgcccagataataaatttgaactcctggaaaggataatgtaaaccacctaacggaacctggcatatagtatgcccagagctctcgcccaccatcccgctacaccctaattaatgatttgttgctaagtcatctgtcttgcccttagactgtgtacccctggggggcatttccttatgtaggctccaccacccctagtcctctgaagtgaaatcagcctcgtaaaacagcaacaacagcatcacctaacacaaactgaatgatcagtgtttagtgtgtatgtttagatagtgcttaattcctagtatgtacaggcaatcccatttttttttcttcatcttaaagttcaggggtccatgtgcaggatcaatgaatcccatttttaatatacccatgcagaacacacatgcaataaaatatatacatacacacatgcatctcaaaattcttagtgtaattttaagctttaaaaacaacaaaattataaaagcaacagacttaacatcatctggaagttcaattatttaaatttcttttacactcagttgatcaattttgaatgcaaaagttttgatttcacatcttttagtccctctcattagaaatgaaaaatgctaaaattccccaaacagaatctggggaaatttcagaagttacgttcactttagctactagaggaatgttttcattttctttctatggcaaagtgttcaatctggaggcagtaaccagtggattctaggcctgtagctctcccaaccctgagtgctgtgcaggtggctggcagcagtggctgctatcaaattttgtctctcttttgtaaactgcaccacacaagagccatcttctgccttggcttgcttctcaccaacacagaactgttctccatggtgtggaggagacataaagtatttcaggaactgtactaccttcttactgccgacagtcacagacaggtacaaccaatataaatgagctcttcatcctgtcctttaaccacccaaatgcagtgttaaaacattcttctggtccttccaccatcctgtacctgcaggatgcttgtatagattaccccacctactcgaatctctgttagttctgttatttcatgtcaggtgacctttaaaagcttgaaaatctgtgtcatgcattagctctcctgggtgaaagctgcttatgttccagtctgccagaagcatggttctcagtaagctaggctattcttcaactgccacgctctcaacaaatttcagataatattggagattaacaaatgcaaaaagacttgcagatgacttataaattataaagccactccaaaaatgcttttgttagctaagattttcaaaccgtacagtacttaatgtttggaataactcatcaaaaaggctgaaattgtgctcactagaatgatcaacaacccgaggagacaaaaaacaactcaataaaaacttaatgaatttatttcctatcagtcttgtcaggttgcattttgaattctatccacagcatgtgatgaaagtacccaaaccataatgtaatcttatgtactacatcaaggatctagtcagcataattttctgggatctggtgtgaaagcacactcctttgtgtctacaatccttccgcaggaagggcctttccccaacgcaatcaatcaatcaatccatcaatcaatcatcagtccagaaaagcctaattgctcacccatcaccagttctgattataattagtgttctataatcatggagcaggaagcacaagatgggaaaggaggggggccaccgaggtcctccgaggcacttggtaatcacgatcagccgttttataccaatagcctagaagccaaacacacaactgctcgctctggttaaattctgttaaaccagtactaataagaatggaagtacaaagcttgaaacaatgatttcttatcctaaaaacagattctgcatgagcagaaaagcagggataagcagagtgaagtgtttgagagtgagaagcattatgcggatggctagaaagaaaacctcaatcgagaatgactcgcaatagccttaaacctgctgctgaaaatgccccctgatgcatatttattaggtctgtcatccaagaggcttgtatgccacagtatttccagccatcattaataggcattaatgaccacagcctttcaacgccactgtggcgcactgcaatgcagctccgagcagctggtggaatcagaacagatggcctgcttcccttcaaggcaggactttctgcaggtgacaacatgactgctaggtgactgacaaa

SEQ ID NO: 9067 - RNA, 1031 nt, Homo sapiens
  source 1..1031: mol_type = other RNA
actggacttggagtcagaagagtggttgtccttgagaagagcagtgactgagagggaacacacaagtggcttctggggcactagcaatgttctgtttcttgatctgctgctggttacacaaatgtattccatttgtgaaaattcatcaagatatatacttgtcatttgtgcatttttctgcatgtatattataaattaattttttaaattgtggtaaaaaaaaaaaccataatgtatacaatttaaaaaatttttaggccgggcgcagtggctcatgcctgtaatcccagcactttgggaggccgaggcgggcggatcaccaggtcaggagaccgagaccatcctggctaacacggtgaaaccccgtctctactaaaaatacaaaaaattagccaggtgtggtggtgggcacctgtagtcccagctattcgggaggctgaggcaggagaatcgcttgaaccagggagttggaggttccagtgagccgagatcgtgccactgcactccagcctgggtgacagagtgagactccgtcaccgcggtcggagcccgggtctcactctcctgccgctgtttcgggccacaccgtgtgtccgtgcctccgcaaaggaatagaagagtgggtcctcgctctctgcggcgcaccgcttgtcccttgacttcctgtccatctacaaagcctatttcatgttttccagaaagaaaacgttttccgtgtctcttgagtcctcatcgccatatgcggggcgggaccgatctatgcaaaagatcgcaagagaaaactgatggagcatcgcccatcatgaggctgctctcccgatggtcactgagttgtgttgtggcactgtctttgtacaaagacaccaatttttgcgaacggtgccactcatgattcaacgctctcatgcctcggtcccagctgctggagcgcagattttcctccaagggttagaagatagaaaactcctcggtaattggcctagaggtggtctgcgaggacgccgggaagcttgtaattggctgtttaattc

SEQ ID NO: 9068 - RNA, 8750 nt, Homo sapiens
  source 1..8750: mol_type = other RNA
actggacttggagtcagaaggccagggtttgagtcttggctctgtcatctgttgagctgggaaaatcagaataagtgcaataggcagagtcacagaggaaggactggttaatttggcctgggatggtcagggaaagcattagaggggtgagaacattttagctagttctcaaagaatgattgggagtttgtcaggtgagtgaggtgagataggggatgtgatgtattctagataaattgaatagtaacaaaaatcatatataatgaaaatgtacaacatcttcagggggtagtgagttacctgggaaggccagagctccagtgtatgggaaaactgttcaggatattgttgaaatcaggttgtgaaggcccttgaatactttttgaaggggtttggacttcaatctgctgccagaggtgctccaacttcagtttttaatcagatgggtcaaaaagtcagattcatattttacatgctgctggcagcagctctgagatgacttggagggagtgggcccagaagggagagaggaagacagaggattttttcctagtgcaggtgtgagatgagacactattgtttttcctgtctattttaataaagagtcattcatacttctgctgcagggcaagtttagtgagcatgcatggacaggtaggagtaagagactgtcctagatggtaggtgacaactggctggttatctggctgtgtcatgggtacctgagaagttccaggggagcaggctggagaggcacccctgggggtttctggtacaaggtttcaaaggcctcagtgatgagggcccagacatctttctaaggccgggatgccggccccttgggggagtcccttgatccagatagcatgacagagcactcagttttctgtgtgtgtgggcctttgaacctcttcaaagtcaagaggattttctctctgccacagacagaatattagtcctcatttatgtgcttttgtcattagaatacacgaagtatctattcttgtaaaaacctcagttgcacttggctggaagccactgttgttacatttgttggacacagctggtactctatcaagcctgaagaataaaactagtgataatcatgattccaatcagagttaattgatggagaaataatattattctatgtaacattaaaggaaaagaccactggtctggccatgtgatatggtagtgaagtgggtatttgttgtagggttatgtagaggttgaatggtgtcactagggagagtgaaaggtctcttgtggtaactagatgggaaaaggaacaaagccaatatgaacccccacaaatttatgactttgtatttacatgagaacaaaaaagactaagtagaaggaatacggggccaactggaaatgctcctgtcctacagttgttattgacttgagtgagtcacccaagcttttgtgcttgagatatcacatctgccatttaaggggaatagtttctattacttctctactgaaaaaaatacatgaagtgtcattccaatgctttcagtggtaaggattagaaatactatcaaaaataggcatccatgccaatccagccagtgagagagcactgttaacttctgtaagtaagaatagtcttgatctgtgaagtgggattagtacttacctttctggattgtcatgaaggtaaagtgtgatgagattcgcaaagtgaccagcacacctggcatctatctatatctgtagcagtatatctaatgtgtgtgtgtacacacacaagtataatagttggatgcttttattcccactccaattacatgctttcttcagtgagcccagttccaattcatatgcgggtacttgctgttttcatacccacatgttaacactgacattgacctgttctctttgaattgcaagaactggaaccaggtaggaatgtcatgggctgagtagaaagctatacgagttacaatggaaattactttgagcttacacgtcctataatcccagattaaccatatcttccaatttggagagtaattccaatataaatcactgttatggagtgctaggttgtggattactacccttttggaattaaacctaaaggcaggaattctttaggttatctctggaaactaacttcccattataaggcctagactctctactcagggcttgccagtcaatggttccccttgcctacaggttaaagtccaaagtccttggcatgacatataaggctatacatggcaagatcccagctttcctgccaccctcagctatcattaattttatcttcacatccagtactgcagccatatcagaccacttacaatttctcaaacgtcttaggtaattttaatctctgcagatgcttggaatgttctcccaccctctactggccttaccttcctacccaatctacctcatatgttaccacatcagagcatgagtccacctcatctgaatggtaactctctctcttatgcctccagtatagcttgtacatacgtccttcatagcagttacctcactgattttaatcatttgcatatttatttttctctgagttatgagctcttggaggacagagaccatatctgtagaaattggcttcatatcacctgattattcttttagaattaagtgtcatgaaataaaagctttctttgtatcttactgtattgcccacccctttcctattttcttggcaccagaaaactcagaacaaaatttaactgtagcgtacaggaattgatgatacatatcttgacattgcagtctttctagaccttttttgtctcaattttatattatctatgaatatttccaacttttattgtatatattcaggtagtcatcttcaagtcatttgaagagtgacttgtagattacactaaaaatgtcatctgatctttcaagtttccttgaaccttttcaaggtacggagcatctggcactctgccctggtttctttgtgattttgatttgcatttccctgatagctattgatattgacatttttcacgtgcttattggttggccattcatatgtcttctttggagaaatttctatttaaatcatttgctcatggaaaaaaatgggctgtttgtctttattgagttgtaagagttctgtatatattttgggtgtaagtatcttactaaatatgcaattttcaaaatttttctctcagtctgtagggttatctttttactttcttaaaaatatcccttgaagcagaaaagtttttgattttgatgaagtccaacctagccatcttttatcacctgtgctttaggtgtctaatttgaagagtcattccctaatccgagatcatgaagattgaattttgtagttgttttgaaaagagttttgtaatttagctcttacatttagatctataatacactttgagttaatttgtgtctattgtgaagtcagggtgcaaattcattcttttgcatgtgatattcagttgtccagcactatttgttaaagattattctttgcccactgaattgtcttgcctatttactgaaaatcgattgaacataaatgtgaggatttactggactcttaattctattctgttgattaatatgtttatccctataccagtaccacaccattatgattactgtcgctttgtagtatgttctggaattgggaagtgtgaatccatcaactttgttattctttttcaagattgttatagtgattctggatcccttgcatttttatatacatgttagggtcaccttgtgaatttctgtaaaaacaccagaagagttttgttaagaattgcattaagtttgtacattaatatgggaagtattgccatcttaacgatattaaatcctccaattcataagcatggtgtatctttccatttattttaatcttcagtatcactcaacagtgttttgtagtttttagcatatacattttatacttaaattgttaaatctattcctaaaaattttattccttttgatgttatttataaatagaattttcttaattttattttggtttttcattgttaatatatagaaatgcaatcgatttttctatactgatcttgtatccagcaaacttgctgaacccatttattagttctaatagcttttttttttgttttttgtcgataccttgggattttctacataggagattttcacatctgagagtgaaagaagaccatttgattctttacaatttagtatgatgttagctgtaagtttctggtagtttgaggaagttaatttttgttcctggtttaagcgttttcttctttttttgtttaatcatgagtgttggagtttatccattattttatgcatctattgaagtaattgtgatttttttctttattgttgtggcatattatataaattgattttcagatgttaaaccaatcttgaattcttggaagaaatctttcttagttgtggtacaattttttatttgtttcaggattcatcttggagttttgcatctatattcataaaggatagggatgcataaaggtgtgcagttctctttttctcatgcctttgtctggcattggtatcagggtaatagtgaactcatagaatgagttcccctttcttctattttctaaaagagtttataaacaattggtattaattcttctttaaatatttgggagaatttaccagtggaagccatctaggcctgaatctttctttgtgggaagtttttatttactaattcaatctttttacctgttataggtctatttagattttctatttcttgagttagtttcaataatttgtgtctttctagggatttgtccatatcatatagtttatttaatttgttagcaatagaggttttttttttttacgttttatcccccttgaattctttttatctgtaaagttagtagtcaagtttcttctttcttgcctgatgtgagtaatttgagtcctccttcttttttgctaaagtttcgctaaagatttgtcaattttgttcaagaaccaactgttgctttatgtattttattttttatttcatttatttctactgaaattttattattttctcctttttgcttgctttcagtttcatttgttcttttatagtttcataaattgaaaggttagattattagagatattttttaaagaaataagcatttattgctataaatttagctctaatgctgctttaacttcctcccatggttttttttgtatgctgtatttttattttcattcatctcaagtatcttctaattttccttgtgatatttttttcccttgacctattggttatttatgaacgtgttgcttaatttccacatatttgtgtattccccacatttcttttagttattgatttctaaatctgtgggcatagagcctaatttacatgatttcagtcttttattatctattgtggcttattttatggcctagcacatcatatatttctgtggaatgttccgtatgcacttcagaagaatgtattttctgctgttgttgggtggagttttctatagatgtgtgttgattctacttggtttacaatgtttttcaagtctctgtatcccagttggttttctgcccagtttttctctttattgttggaagtgaggtattccagtcctcaactattattgttgaattgtctatctttcccttcaattttgtcagttgttgctttacgtattttgggattttgttattaggtacatacatacttgttattcttgttacatcttccttattgaataaattgtcatcacttaaaatgtccctcttcatctctaataagtttttgtcttacagactattttatctagtattagtatagctgccccaactctgtatgattgctgttttcatggtatatctttttctatccttttacttttcttttaaaataattttaaaaattaatttacatacactaaaatgcagagattttaagtgctcagttcaatgactgttgacaattatacacagctatgtatccacccccaaacaagatataaaccatatataatatttcatacagttttctcatgcccctttccagtcaatccccatctccttcctgtaacaggcaagtgctttctgatcataatgatctttttaaaatcatagtatattcatttgtctgttctaggttttatggtaatgaaaccaaacaggaggtattcttttgtgtctggctgctttctttccatattatgtttttaagattcatttatattgttgcatttactttttattgctgagtaatagcaaatgaatataacctagtgcagtccaaggtcagccctcttcagaaggactctgcaaaggttcactccactttccagatgataaaattgagaaaccttcaggagcattaattcttttgttactgcctctgaattaacatgtgagagaagctctcagagcttggaggaggatgactacatgatgagtttggagccaaaccctctgctccttacctcacgtatcttcctagtcatatacctaatatctggtttagtgtaaaaaatgaagaattaagaggcagaaaatacactaccctgttctacttccatcactagttcaacatatgtcatccactttctggatttttttctcctttgagtaatgaagagcttgatttggtcatctctaggatgcctttcatctctgatatactatttagttgttggtcaatgacatctaagtatgaattcgtttatgaaacacaaaagcaattttaactatgcttctctgcaatggtaaccattctcccaagagaaaggcaacaaaaagtgaagtgattcaggaatcctaattttgcccaccccacagttacacacagcacttggcatgtatgtaaaagtagcatggaaagcaccagatatgactggctgtgatacaagttctggtctgcacttccacgtacaagatgtccatgcttgccttgatctcttattcccttttgagccatagtttcatagctagttaatggcagagctgagattagaatccaggtctccttattctctgggcagtgactttcttccacatccatctttcttccttactttcacatctggtgccttacagatcctcagcacagccaagaactatacccattaggatagaagtgggaggagtagatggatttgcaggggagggttttgcagcatcctcaaacttctctcggagctggtaggctccaaagagattgagacttcgaggacagttggccattctcaaattaaacatagtacccacattcatgtgtggaaatgttcaatatttcttaggctttgaacttgataacgtagtggactatcagccctttttaatatttcttaatcactggttaatgtgaattctcagaactgagaggttcttcttgtgtagctgatttccgctgagttccttcttttttctaattttggtatgatggcactgtgtctaatgaagcaagtcaaataaacggcagattctgttccccgaagccctcttcatcctggaacattaactgtctaatttgttcatgggaagacccagctgttagcaggcagcctgcgggccccaaagcaaatgaggagaagccttcctgtgaacttcagaacacatgctggggtgggggctgtggggagacattttgtttatcactcatttaaagtatgttgctcccaaataaatggctgtaaatggagatgaagggataagacttgtgactaatttctctggggagcctaagtatctccactcctgaccccagtgtgctgcctcccccatcttcccattgtaagactcacagcagctttatgacaaggtgggtgtttatgatccagttcaggatggggactaacccagtcctccctggtggaggcattctttccatgacggggctgacgctctgccaataggatcccagtgagctcagggaacagtgtcaggttgattcagctgaggaagtcacggccttgatttagccttaaaaggctgaggttccggtggaagcgagtctgtctcagcgtgaaagcccaaggctctgagcattcccagatgacatctgtgatttttccaacacacatttggcctccttggttccttgcagtgctttggttgtgcaatcaccacttggcaggttcttcgtccagtgaaatctgtacattttcagctctgacatctcaaaaataatcattggagcattttttttatcagagtggtttatcgtaaaacaaccactcccaccgacatttcttgtaaccagtgctaggagagtgacgacttagaaggccttttgaggaaggagtagtggaagaagggctggtttcggaattgaacacaccagggttccaattctagcttccttttattacatgttgccggaccttaggccttcaggggctcagtttcatcttctataaagtagagaaaatagtatataccttgcaatgtagttgtgaggattagatatcaaatctatcattagattagttcatcagatggactcagtacactttgtatgaatatatgagtgggatgtgtgtgtgttgtgtagtgttggtcctaggttagaggtgagagtggttataagtttagtgtatatagagggaatatcagctctctttttagccctcaataaatcacaaacatgcacatacacactgcacgtgtgcacacattcttgaaaacctcagcttttttctttttgatgttgagatagctaaagattcctttctttagattttttttta

SEQ ID NO: 9069 - RNA, 8955 nt, Homo sapiens
  source 1..8955: mol_type = other RNA
actggacttggagtcagaaggccagggtttgagtcttggctctgtcatctgttgagctgggaaaatcagaataagtgcaataggcagagtcacagaggaaggactggttaatttggcctgggatggtcagggaaagcattagaggggtgagaacattttagctagttctcaaagaatgattgggagtttgtcaggtgagtgaggtgagataggggatgtgatgtattctagataaattgaatagtaacaaaaatcatatataatgaaaatgtacaacatcttcagggggtagtgagttacctgggaaggccagagctccagtgtatgggaaaactgttcaggatattgttgaaatcaggttgtgaaggcccttgaatactttttgaaggggtttggacttcaatctgctgccagaggtgctccaacttcagtttttaatcagatgggtcaaaaagtcagattcatattttacatgctgctggcagcagctctgagatgacttggagggagtgggcccagaagggagagaggaagacagaggattttttcctagtgcaggtgtgagatgagacactattgtttttcctgtctattttaataaagagtcattcatacttctgctgcagggcaagtttagtgagcatgcatggacaggtaggagtaagagactgtcctagatggtaggtgacaactggctggttatctggctgtgtcatgggtacctgagaagttccaggggagcaggctggagaggcacccctgggggtttctggtacaaggtttcaaaggcctcagtgatgagggcccagacatctttctaaggccgggatgccggccccttgggggagtcccttgatccagatagcatgacagagcactcagttttctgtgtgtgtgggcctttgaacctcttcaaagtcaagaggattttctctctgccacagacagaatattagtcctcatttatgtgcttttgtcattagaatacacgaagtatctattcttgtaaaaacctcagttgcacttggctggaagccactgttgttacatttgttggacacagctggtactctatcaagcctgaagaataaaactagtgataatcatgattccaatcagagttaattgatggagaaataatattattctatgtaacattaaaggaaaagaccactggtctggccatgtgatatggtagtgaagtgggtatttgttgtagggttatgtagaggttgaatggtgtcactagggagagtgaaaggtctcttgtggtaactagatgggaaaaggaacaaagccaatatgaacccccacaaatttatgactttgtatttacatgagaacaaaaaagactaagtagaaggaatacggggccaactggaaatgctcctgtcctacagttgttattgacttgagtgagtcacccaagcttttgtgcttgagatatcacatctgccatttaaggggaatagtttctattacttctctactgaaaaaaatacatgaagtgtcattccaatgctttcagtggtaaggattagaaatactatcaaaaataggcatccatgccaatccagccagtgagagagcactgttaacttctgtaagtaagaatagtcttgatctgtgaagtgggattagtacttacctttctggattgtcatgaaggtaaagtgtgatgagattcgcaaagtgaccagcacacctggcatctatctatatctgtagcagtatatctaatgtgtgtgtgtacacacacaagtataatagttggatgcttttattcccactccaattacatgctttcttcagtgagcccagttccaattcatatgcgggtacttgctgttttcatacccacatgttaacactgacattgacctgttctctttgaattgcaagaactggaaccaggtaggaatgtcatgggctgagtagaaagctatacgagttacaatggaaattactttgagcttacacgtcctataatcccagattaaccatatcttccaatttggagagtaattccaatataaatcactgttatggagtgctaggttgtggattactacccttttggaattaaacctaaaggcaggaattctttaggttatctctggaaactaacttcccattataaggcctagactctctactcagggcttgccagtcaatggttccccttgcctacaggttaaagtccaaagtccttggcatgacatataaggctatacatggcaagatcccagctttcctgccaccctcagctatcattaattttatcttcacatccagtactgcagccatatcagaccacttacaatttctcaaacgtcttaggtaattttaatctctgcagatgcttggaatgttctcccaccctctactggccttaccttcctacccaatctacctcatatgttaccacatcagagcatgagtccacctcatctgaatggtaactctctctcttatgcctccagtatagcttgtacatacgtccttcatagcagttacctcactgattttaatcatttgcatatttatttttctctgagttatgagctcttggaggacagagaccatatctgtagaaattggcttcatatcacctgattattcttttagaattaagtgtcatgaaataaaagctttctttgtatcttactgtattgcccacccctttcctattttcttggcaccagaaaactcagaacaaaatttaactgtagcgtacaggaattgatgatacatatcttgacattgcagtctttctagaccttttttgtctcaattttatattatctatgaatatttccaacttttattgtatatattcaggtagtcatcttcaagtcatttgaagagtgacttgtagattacactaaaaatgtcatctgatctttcaagtttccttgaaccttttcaaggtacggagcatctggcactctgccctggtttctttgtgattttgatttgcatttccctgatagctattgatattgacatttttcacgtgcttattggttggccattcatatgtcttctttggagaaatttctatttaaatcatttgctcatggaaaaaaatgggctgtttgtctttattgagttgtaagagttctgtatatattttgggtgtaagtatcttactaaatatgcaattttcaaaatttttctctcagtctgtagggttatctttttactttcttaaaaatatcccttgaagcagaaaagtttttgattttgatgaagtccaacctagccatcttttatcacctgtgctttaggtgtctaatttgaagagtcattccctaatccgagatcatgaagattgaattttgtagttgttttgaaaagagttttgtaatttagctcttacatttagatctataatacactttgagttaatttgtgtctattgtgaagtcagggtgcaaattcattcttttgcatgtgatattcagttgtccagcactatttgttaaagattattctttgcccactgaattgtcttgcctatttactgaaaatcgattgaacataaatgtgaggatttactggactcttaattctattctgttgattaatatgtttatccctataccagtaccacaccattatgattactgtcgctttgtagtatgttctggaattgggaagtgtgaatccatcaactttgttattctttttcaagattgttatagtgattctggatcccttgcatttttatatacatgttagggtcaccttgtgaatttctgtaaaaacaccagaagagttttgttaagaattgcattaagtttgtacattaatatgggaagtattgccatcttaacgatattaaatcctccaattcataagcatggtgtatctttccatttattttaatcttcagtatcactcaacagtgttttgtagtttttagcatatacattttatacttaaattgttaaatctattcctaaaaattttattccttttgatgttatttataaatagaattttcttaattttattttggtttttcattgttaatatatagaaatgcaatcgatttttctatactgatcttgtatccagcaaacttgctgaacccatttattagttctaatagcttttttttttgttttttgtcgataccttgggattttctacataggagattttcacatctgagagtgaaagaagaccatttgattctttacaatttagtatgatgttagctgtaagtttctggtagtttgaggaagttaatttttgttcctggtttaagcgttttcttctttttttgtttaatcatgagtgttggagtttatccattattttatgcatctattgaagtaattgtgatttttttctttattgttgtggcatattatataaattgattttcagatgttaaaccaatcttgaattcttggaagaaatctttcttagttgtggtacaattttttatttgtttcaggattcatcttggagttttgcatctatattcataaaggatagggatgcataaaggtgtgcagttctctttttctcatgcctttgtctggcattggtatcagggtaatagtgaactcatagaatgagttcccctttcttctattttctaaaagagtttataaacaattggtattaattcttctttaaatatttgggagaatttaccagtggaagccatctaggcctgaatctttctttgtgggaagtttttatttactaattcaatctttttacctgttataggtctatttagattttctatttcttgagttagtttcaataatttgtgtctttctagggatttgtccatatcatatagtttatttaatttgttagcaatagaggttttttttttttacgttttatcccccttgaattctttttatctgtaaagttagtagtcaagtttcttctttcttgcctgatgtgagtaatttgagtcctccttcttttttgctaaagtttcgctaaagatttgtcaattttgttcaagaaccaactgttgctttatgtattttattttttatttcatttatttctactgaaattttattattttctcctttttgcttgctttcagtttcatttgttcttttatagtttcataaattgaaaggttagattattagagatattttttaaagaaataagcatttattgctataaatttagctctaatgctgctttaacttcctcccatggttttttttgtatgctgtatttttattttcattcatctcaagtatcttctaattttccttgtgatatttttttcccttgacctattggttatttatgaacgtgttgcttaatttccacatatttgtgtattccccacatttcttttagttattgatttctaaatctgtgggcatagagcctaatttacatgatttcagtcttttattatctattgtggcttattttatggcctagcacatcatatatttctgtggaatgttccgtatgcacttcagaagaatgtattttctgctgttgttgggtggagttttctatagatgtgtgttgattctacttggtttacaatgtttttcaagtctctgtatcccagttggttttctgcccagtttttctctttattgttggaagtgaggtattccagtcctcaactattattgttgaattgtctatctttcccttcaattttgtcagttgttgctttacgtattttgggattttgttattaggtacatacatacttgttattcttgttacatcttccttattgaataaattgtcatcacttaaaatgtccctcttcatctctaataagtttttgtcttacagactattttatctagtattagtatagctgccccaactctgtatgattgctgttttcatggtatatctttttctatccttttacttttcttttaaaataattttaaaaattaatttacatacactaaaatgcagagattttaagtgctcagttcaatgactgttgacaattatacacagctatgtatccacccccaaacaagatataaaccatatataatatttcatacagttttctcatgcccctttccagtcaatccccatctccttcctgtaacaggcaagtgctttctgatcataatgatctttttaaaatcatagtatattcatttgtctgttctaggttttatggtaatgaaaccaaacaggaggtattcttttgtgtctggctgctttctttccatattatgtttttaagattcatttatattgttgcatttactttttattgctgagtaatagcaaatgaatataacctagtgcagtccaaggtcagccctcttcagaaggactctgcaaaggttcactccactttccagatgataaaattgagaaaccttcaggagcattaattcttttgttactgcctctgaattaacatgtgagagaagctctcagagcttggaggaggatgactacatgatgagtttggagccaaaccctctgctccttacctcacgtatcttcctagtcatatacctaatatctggtttagtgtaaaaaatgaagaattaagaggcagaaaatacactaccctgttctacttccatcactagttcaacatatgtcatccactttctggatttttttctcctttgagtaatgaagagcttgatttggtcatctctaggatgcctttcatctctgatatactatttagttgttggtcaatgacatctaagtatgaattcgtttatgaaacacaaaagcaattttaactatgcttctctgcaatggtaaccattctcccaagagaaaggcaacaaaaagtgaagtgattcaggaatcctaattttgcccaccccacagttacacacagcacttggcctcacttattaaggaaaacagaaaacaaaaaacaaaaagtctccccattagcagggcaggaaggatacagtcccttaggaaaccaagaaaccaaatgacctgacaaatgaattaagattgtcaatgtctgctgcaccttttaggtttggaagttacaaagtaaagagtttagactaaactagaagaggatcaaatttaaggatacatgtatgtaaaagtagcatggaaagcaccagatatgactggctgtgatacaagttctggtctgcacttccacgtacaagatgtccatgcttgccttgatctcttattcccttttgagccatagtttcatagctagttaatggcagagctgagattagaatccaggtctccttattctctgggcagtgactttcttccacatccatctttcttccttactttcacatctggtgccttacagatcctcagcacagccaagaactatacccattaggatagaagtgggaggagtagatggatttgcaggggagggttttgcagcatcctcaaacttctctcggagctggtaggctccaaagagattgagacttcgaggacagttggccattctcaaattaaacatagtacccacattcatgtgtggaaatgttcaatatttcttaggctttgaacttgataacgtagtggactatcagccctttttaatatttcttaatcactggttaatgtgaattctcagaactgagaggttcttcttgtgtagctgatttccgctgagttccttcttttttctaattttggtatgatggcactgtgtctaatgaagcaagtcaaataaacggcagattctgttccccgaagccctcttcatcctggaacattaactgtctaatttgttcatgggaagacccagctgttagcaggcagcctgcgggccccaaagcaaatgaggagaagccttcctgtgaacttcagaacacatgctggggtgggggctgtggggagacattttgtttatcactcatttaaagtatgttgctcccaaataaatggctgtaaatggagatgaagggataagacttgtgactaatttctctggggagcctaagtatctccactcctgaccccagtgtgctgcctcccccatcttcccattgtaagactcacagcagctttatgacaaggtgggtgtttatgatccagttcaggatggggactaacccagtcctccctggtggaggcattctttccatgacggggctgacgctctgccaataggatcccagtgagctcagggaacagtgtcaggttgattcagctgaggaagtcacggccttgatttagccttaaaaggctgaggttccggtggaagcgagtctgtctcagcgtgaaagcccaaggctctgagcattcccagatgacatctgtgatttttccaacacacatttggcctccttggttccttgcagtgctttggttgtgcaatcaccacttggcaggttcttcgtccagtgaaatctgtacattttcagctctgacatctcaaaaataatcattggagcattttttttatcagagtggtttatcgtaaaacaaccactcccaccgacatttcttgtaaccagtgctaggagagtgacgacttagaaggccttttgaggaaggagtagtggaagaagggctggtttcggaattgaacacaccagggttccaattctagcttccttttattacatgttgccggaccttaggccttcaggggctcagtttcatcttctataaagtagagaaaatagtatataccttgcaatgtagttgtgaggattagatatcaaatctatcattagattagttcatcagatggactcagtacactttgtatgaatatatgagtgggatgtgtgtgtgttgtgtagtgttggtcctaggttagaggtgagagtggttataagtttagtgtatatagagggaatatcagctctctttttagccctcaataaatcacaaacatgcacatacacactgcacgtgtgcacacattcttgaaaacctcagcttttttctttttgatgttgagatagctaaagattcctttctttagattttttttta

SEQ ID NO: 9070 - RNA, 9102 nt, Homo sapiens
  source 1..9102: mol_type = other RNA
actggacttggagtcagaaggccagggtttgagtcttggctctgtcatctgttgagctgggaaaatcagaataagtgcaataggcagagtcacagaggaaggactggttaatttggcctgggatggtcagggaaagcattagaggggtgagaacattttagctagttctcaaagaatgattgggagtttgtcaggtgagtgaggtgagataggggatgtgatgtattctagataaattgaatagtaacaaaaatcatatataatgaaaatgtacaacatcttcagggggtagtgagttacctgggaaggccagagctccagtgtatgggaaaactgttcaggatattgttgaaatcaggttgtgaaggcccttgaatactttttgaaggggtttggacttcaatctgctgccagaggtgctccaacttcagtttttaatcagatgggtcaaaaagtcagattcatattttacatgctgctggcagcagctctgagatgacttggagggagtgggcccagaagggagagaggaagacagaggattttttcctagtgcaggtgtgagatgagacactattgtttttcctgtctattttaataaagagtcattcatacttctgctgcagggcaagtttagtgagcatgcatggacaggtaggagtaagagactgtcctagatggtaggtgacaactggctggttatctggctgtgtcatgggtacctgagaagttccaggggagcaggctggagaggcacccctgggggtttctggtacaaggtttcaaaggcctcagtgatgagggcccagacatctttctaaggccgggatgccggccccttgggggagtcccttgatccagatagcatgacagagcactcagttttctgtgtgtgtgggcctttgaacctcttcaaagtcaagaggattttctctctgccacagacagaatattagtcctcatttatgtgcttttgtcattagaatacacgaagtatctattcttgtaaaaacctcagttgcacttggctggaagccactgttgttacatttgttggacacagctggtactctatcaagcctgaagaataaaactagtgataatcatgattccaatcagagttaattgatggagaaataatattattctatgtaacattaaaggaaaagaccactggtctggccatgtgatatggtagtgaagtgggtatttgttgtagggttatgtagaggttgaatggtgtcactagggagagtgaaaggtctcttgtggtaactagatgggaaaaggaacaaagccaatatgaacccccacaaatttatgactttgtatttacatgagaacaaaaaagactaagtagaaggaatacggggccaactggaaatgctcctgtcctacagttgttattgacttgagtgagtcacccaagcttttgtgcttgagatatcacatctgccatttaaggggaatagtttctattacttctctactgaaaaaaatacatgaagtgtcattccaatgctttcagtggtaaggattagaaatactatcaaaaataggcatccatgccaatccagccagtgagagagcactgttaacttctgtaagtaagaatagtcttgatctgtgaagtgggattagtacttacctttctggattgtcatgaaggtaaagtgtgatgagattcgcaaagtgaccagcacacctggcatctatctatatctgtagcagtatatctaatgtgtgtgtgtacacacacaagtataatagttggatgcttttattcccactccaattacatgctttcttcagtgagcccagttccaattcatatgcgggtacttgctgttttcatacccacatgttaacactgacattgacctgttctctttgaattgcaagaactggaaccaggtaggaatgtcatgggctgagtagaaagctatacgagttacaatggaaattactttgagcttacacgtcctataatcccagattaaccatatcttccaatttggagagtaattccaatataaatcactgttatggagtgctaggttgtggattactacccttttggaattaaacctaaaggcaggaattctttaggttatctctggaaactaacttcccattataaggcctagactctctactcagggcttgccagtcaatggttccccttgcctacaggttaaagtccaaagtccttggcatgacatataaggctatacatggcaagatcccagctttcctgccaccctcagctatcattaattttatcttcacatccagtactgcagccatatcagaccacttacaatttctcaaacgtcttaggtaattttaatctctgcagatgcttggaatgttctcccaccctctactggccttaccttcctacccaatctacctcatatgttaccacatcagagcatgagtccacctcatctgaatggtaactctctctcttatgcctccagtatagcttgtacatacgtccttcatagcagttacctcactgattttaatcatttgcatatttatttttctctgagttatgagctcttggaggacagagaccatatctgtagaaattggcttcatatcacctgattattcttttagaattaagtgtcatgaaataaaagctttctttgtatcttactgtattgcccacccctttcctattttcttggcaccagaaaactcagaacaaaatttaactgtagcgtacaggaattgatgatacatatcttgacattgcagtctttctagaccttttttgtctcaattttatattatctatgaatatttccaacttttattgtatatattcaggtagtcatcttcaagtcatttgaagagtgacttgtagattacactaaaaatgtcatctgatctttcaagtttccttgaaccttttcaaggtacggagcatctggcactctgccctggtttctttgtgattttgatttgcatttccctgatagctattgatattgacatttttcacgtgcttattggttggccattcatatgtcttctttggagaaatttctatttaaatcatttgctcatggaaaaaaatgggctgtttgtctttattgagttgtaagagttctgtatatattttgggtgtaagtatcttactaaatatgcaattttcaaaatttttctctcagtctgtagggttatctttttactttcttaaaaatatcccttgaagcagaaaagtttttgattttgatgaagtccaacctagccatcttttatcacctgtgctttaggtgtctaatttgaagagtcattccctaatccgagatcatgaagattgaattttgtagttgttttgaaaagagttttgtaatttagctcttacatttagatctataatacactttgagttaatttgtgtctattgtgaagtcagggtgcaaattcattcttttgcatgtgatattcagttgtccagcactatttgttaaagattattctttgcccactgaattgtcttgcctatttactgaaaatcgattgaacataaatgtgaggatttactggactcttaattctattctgttgattaatatgtttatccctataccagtaccacaccattatgattactgtcgctttgtagtatgttctggaattgggaagtgtgaatccatcaactttgttattctttttcaagattgttatagtgattctggatcccttgcatttttatatacatgttagggtcaccttgtgaatttctgtaaaaacaccagaagagttttgttaagaattgcattaagtttgtacattaatatgggaagtattgccatcttaacgatattaaatcctccaattcataagcatggtgtatctttccatttattttaatcttcagtatcactcaacagtgttttgtagtttttagcatatacattttatacttaaattgttaaatctattcctaaaaattttattccttttgatgttatttataaatagaattttcttaattttattttggtttttcattgttaatatatagaaatgcaatcgatttttctatactgatcttgtatccagcaaacttgctgaacccatttattagttctaatagcttttttttttgttttttgtcgataccttgggattttctacataggagattttcacatctgagagtgaaagaagaccatttgattctttacaatttagtatgatgttagctgtaagtttctggtagtttgaggaagttaatttttgttcctggtttaagcgttttcttctttttttgtttaatcatgagtgttggagtttatccattattttatgcatctattgaagtaattgtgatttttttctttattgttgtggcatattatataaattgattttcagatgttaaaccaatcttgaattcttggaagaaatctttcttagttgtggtacaattttttatttgtttcaggattcatcttggagttttgcatctatattcataaaggatagggatgcataaaggtgtgcagttctctttttctcatgcctttgtctggcattggtatcagggtaatagtgaactcatagaatgagttcccctttcttctattttctaaaagagtttataaacaattggtattaattcttctttaaatatttgggagaatttaccagtggaagccatctaggcctgaatctttctttgtgggaagtttttatttactaattcaatctttttacctgttataggtctatttagattttctatttcttgagttagtttcaataatttgtgtctttctagggatttgtccatatcatatagtttatttaatttgttagcaatagaggttttttttttttacgttttatcccccttgaattctttttatctgtaaagttagtagtcaagtttcttctttcttgcctgatgtgagtaatttgagtcctccttcttttttgctaaagtttcgctaaagatttgtcaattttgttcaagaaccaactgttgctttatgtattttattttttatttcatttatttctactgaaattttattattttctcctttttgcttgctttcagtttcatttgttcttttatagtttcataaattgaaaggttagattattagagatattttttaaagaaataagcatttattgctataaatttagctctaatgctgctttaacttcctcccatggttttttttgtatgctgtatttttattttcattcatctcaagtatcttctaattttccttgtgatatttttttcccttgacctattggttatttatgaacgtgttgcttaatttccacatatttgtgtattccccacatttcttttagttattgatttctaaatctgtgggcatagagcctaatttacatgatttcagtcttttattatctattgtggcttattttatggcctagcacatcatatatttctgtggaatgttccgtatgcacttcagaagaatgtattttctgctgttgttgggtggagttttctatagatgtgtgttgattctacttggtttacaatgtttttcaagtctctgtatcccagttggttttctgcccagtttttctctttattgttggaagtgaggtattccagtcctcaactattattgttgaattgtctatctttcccttcaattttgtcagttgttgctttacgtattttgggattttgttattaggtacatacatacttgttattcttgttacatcttccttattgaataaattgtcatcacttaaaatgtccctcttcatctctaataagtttttgtcttacagactattttatctagtattagtatagctgccccaactctgtatgattgctgttttcatggtatatctttttctatccttttacttttcttttaaaataattttaaaaattaatttacatacactaaaatgcagagattttaagtgctcagttcaatgactgttgacaattatacacagctatgtatccacccccaaacaagatataaaccatatataatatttcatacagttttctcatgcccctttccagtcaatccccatctccttcctgtaacaggcaagtgctttctgatcataatgatctttttaaaatcatagtatattcatttgtctgttctaggttttatggtaatgaaaccaaacaggaggtattcttttgtgtctggctgctttctttccatattatgtttttaagattcatttatattgttgcatttactttttattgctgagtaatagcaaatgaatataacctagtgcagtccaaggtcagccctcttcagaaggactctgcaaaggttcactccactttccagatgataaaattgagaaaccttcaggagcattaattcttttgttactgcctctgaattaacatgtgagagaagctctcagagcttggaggaggatgactacatgatgagtttggagccaaaccctctgctccttacctcacgtatcttcctagtcatatacctaatatctggtttagtgtaaaaaatgaagaattaagaggcagaaaatacactaccctgttctacttccatcactagttcaacatatgtcatccactttctggatttttttctcctttgagtaatgaagagcttgatttggtcatctctaggatgcctttcatctctgatatactatttagttgttggtcaatgacatctaagtatgaattcgtttatgaaacacaaaagcaattttaactatgcttctctgcaatggtaaccattctcccaagagaaaggcaacaaaaagtgaagtgattcaggaatcctaattttgcccaccccacagttacacacagcacttggcctcacttattaaggaaaacagaaaacaaaaaacaaaaagtctccccattagcagggcaggaaggatacagtcccttaggaaaccaagaaaccaaatgacctgacaaatgaattaagattgtcaatgtctgctgcaccttttaggtttggaagttacaaagtaaagagtttagactaaactagaagaggatcaaatttaaggatacatgtatgtaaaagtagcatggaaagcaccagatatgactggctgtgatacaagttctggtctgcacttccacgtacaagatgtccatgcttgccttgatctcttattcccttttgagccatagtttcatcaagaaggaagagcattgcttgaatggaagcatgtcccagacactttatcactggtgaagagccgagctcattgtctaaacttggctcctcattttaaaaagtaaaaaaacgagttatcaaaatgattagttattcttgagtctcacagctagttaatggcagagctgagattagaatccaggtctccttattctctgggcagtgactttcttccacatccatctttcttccttactttcacatctggtgccttacagatcctcagcacagccaagaactatacccattaggatagaagtgggaggagtagatggatttgcaggggagggttttgcagcatcctcaaacttctctcggagctggtaggctccaaagagattgagacttcgaggacagttggccattctcaaattaaacatagtacccacattcatgtgtggaaatgttcaatatttcttaggctttgaacttgataacgtagtggactatcagccctttttaatatttcttaatcactggttaatgtgaattctcagaactgagaggttcttcttgtgtagctgatttccgctgagttccttcttttttctaattttggtatgatggcactgtgtctaatgaagcaagtcaaataaacggcagattctgttccccgaagccctcttcatcctggaacattaactgtctaatttgttcatgggaagacccagctgttagcaggcagcctgcgggccccaaagcaaatgaggagaagccttcctgtgaacttcagaacacatgctggggtgggggctgtggggagacattttgtttatcactcatttaaagtatgttgctcccaaataaatggctgtaaatggagatgaagggataagacttgtgactaatttctctggggagcctaagtatctccactcctgaccccagtgtgctgcctcccccatcttcccattgtaagactcacagcagctttatgacaaggtgggtgtttatgatccagttcaggatggggactaacccagtcctccctggtggaggcattctttccatgacggggctgacgctctgccaataggatcccagtgagctcagggaacagtgtcaggttgattcagctgaggaagtcacggccttgatttagccttaaaaggctgaggttccggtggaagcgagtctgtctcagcgtgaaagcccaaggctctgagcattcccagatgacatctgtgatttttccaacacacatttggcctccttggttccttgcagtgctttggttgtgcaatcaccacttggcaggttcttcgtccagtgaaatctgtacattttcagctctgacatctcaaaaataatcattggagcattttttttatcagagtggtttatcgtaaaacaaccactcccaccgacatttcttgtaaccagtgctaggagagtgacgacttagaaggccttttgaggaaggagtagtggaagaagggctggtttcggaattgaacacaccagggttccaattctagcttccttttattacatgttgccggaccttaggccttcaggggctcagtttcatcttctataaagtagagaaaatagtatataccttgcaatgtagttgtgaggattagatatcaaatctatcattagattagttcatcagatggactcagtacactttgtatgaatatatgagtgggatgtgtgtgtgttgtgtagtgttggtcctaggttagaggtgagagtggttataagtttagtgtatatagagggaatatcagctctctttttagccctcaataaatcacaaacatgcacatacacactgcacgtgtgcacacattcttgaaaacctcagcttttttctttttgatgttgagatagctaaagattcctttctttagattttttttta

SEQ ID NO: 9071 - RNA, 9004 nt, Homo sapiens
  source 1..9004: mol_type = other RNA
actggacttggagtcagaaggccagggtttgagtcttggctctgtcatctgttgagctgggaaaatcagaataagtgcaataggcagagtcacagaggaaggactggttaatttggcctgggatggtcagggaaagcattagaggggtgagaacattttagctagttctcaaagaatgattgggagtttgtcaggtgagtgaggtgagataggggatgtgatgtattctagataaattgaatagtaacaaaaatcatatataatgaaaatgtacaacatcttcagggggtagtgagttacctgggaaggccagagctccagtgtatgggaaaactgttcaggatattgttgaaatcaggttgtgaaggcccttgaatactttttgaaggggtttggacttcaatctgctgccagaggtgctccaacttcagtttttaatcagatgggtcaaaaagtcagattcatattttacatgctgctggcagcagctctgagatgacttggagggagtgggcccagaagggagagaggaagacagaggattttttcctagtgcaggtgtgagatgagacactattgtttttcctgtctattttaataaagagtcattcatacttctgctgcagggcaagtttagtgagcatgcatggacaggtaggagtaagagactgtcctagatggtaggtgacaactggctggttatctggctgtgtcatgggtacctgagaagttccaggggagcaggctggagaggcacccctgggggtttctggtacaaggtttcaaaggcctcagtgatgagggcccagacatctttctaaggccgggatgccggccccttgggggagtcccttgatccagatagcatgacagagcactcagttttctgtgtgtgtgggcctttgaacctcttcaaagtcaagaggattttctctctgccacagacagaatattagtcctcatttatgtgcttttgtcattagaatacacgaagtatctattcttgtaaaaacctcagttgcacttggctggaagccactgttgttacatttgttggacacagctggtactctatcaagcctgaagaataaaactagtgataatcatgattccaatcagagttaattgatggagaaataatattattctatgtaacattaaaggaaaagaccactggtctggccatgtgatatggtagtgaagtgggtatttgttgtagggttatgtagaggttgaatggtgtcactagggagagtgaaaggtctcttgtggtaactagatgggaaaaggaacaaagccaatatgaacccccacaaatttatgactttgtatttacatgagaacaaaaaagactaagtagaaggaatacggggccaactggaaatgctcctgtcctacagttgttattgacttgagtgagtcacccaagcttttgtgcttgagatatcacatctgccatttaaggggaatagtttctattacttctctactgaaaaaaatacatgaagtgtcattccaatgctttcagtggtaaggattagaaatactatcaaaaataggcatccatgccaatccagccagtgagagagcactgttaacttctgtaagtaagaatagtcttgatctgtgaagtgggattagtacttacctttctggattgtcatgaaggtaaagtgtgatgagattcgcaaagtgaccagcacacctggcatctatctatatctgtagcagtatatctaatgtgtgtgtgtacacacacaagtataatagttggatgcttttattcccactccaattacatgctttcttcagtgagcccagttccaattcatatgcgggtacttgctgttttcatacccacatgttaacactgacattgacctgttctctttgaattgcaagaactggaaccaggtaggaatgtcatgggctgagtagaaagctatacgagttacaatggaaattactttgagcttacacgtcctataatcccagattaaccatatcttccaatttggagagtaattccaatataaatcactgttatggagtgctaggttgtggattactacccttttggaattaaacctaaaggcaggaattctttaggttatctctggaaactaacttcccattataaggcctagactctctactcagggcttgccagtcaatggttccccttgcctacaggttaaagtccaaagtccttggcatgacatataaggctatacatggcaagatcccagctttcctgccaccctcagctatcattaattttatcttcacatccagtactgcagccatatcagaccacttacaatttctcaaacgtcttaggtaattttaatctctgcagatgcttggaatgttctcccaccctctactggccttaccttcctacccaatctacctcatatgttaccacatcagagcatgagtccacctcatctgaatggtaactctctctcttatgcctccagtatagcttgtacatacgtccttcatagcagttacctcactgattttaatcatttgcatatttatttttctctgagttatgagctcttggaggacagagaccatatctgtagaaattggcttcatatcacctgattattcttttagaattaagtgtcatgaaataaaagctttctttgtatcttactgtattgcccacccctttcctattttcttggcaccagaaaactcagaacaaaatttaactgtagcgtacaggaattgatgatacatatcttgacattgcagtctttctagaccttttttgtctcaattttatattatctatgaatatttccaacttttattgtatatattcaggtagtcatcttcaagtcatttgaagagtgacttgtagattacactaaaaatgtcatctgatctttcaagtttccttgaaccttttcaaggtacggagcatctggcactctgccctggtttctttgtgattttgatttgcatttccctgatagctattgatattgacatttttcacgtgcttattggttggccattcatatgtcttctttggagaaatttctatttaaatcatttgctcatggaaaaaaatgggctgtttgtctttattgagttgtaagagttctgtatatattttgggtgtaagtatcttactaaatatgcaattttcaaaatttttctctcagtctgtagggttatctttttactttcttaaaaatatcccttgaagcagaaaagtttttgattttgatgaagtccaacctagccatcttttatcacctgtgctttaggtgtctaatttgaagagtcattccctaatccgagatcatgaagattgaattttgtagttgttttgaaaagagttttgtaatttagctcttacatttagatctataatacactttgagttaatttgtgtctattgtgaagtcagggtgcaaattcattcttttgcatgtgatattcagttgtccagcactatttgttaaagattattctttgcccactgaattgtcttgcctatttactgaaaatcgattgaacataaatgtgaggatttactggactcttaattctattctgttgattaatatgtttatccctataccagtaccacaccattatgattactgtcgctttgtagtatgttctggaattgggaagtgtgaatccatcaactttgttattctttttcaagattgttatagtgattctggatcccttgcatttttatatacatgttagggtcaccttgtgaatttctgtaaaaacaccagaagagttttgttaagaattgcattaagtttgtacattaatatgggaagtattgccatcttaacgatattaaatcctccaattcataagcatggtgtatctttccatttattttaatcttcagtatcactcaacagtgttttgtagtttttagcatatacattttatacttaaattgttaaatctattcctaaaaattttattccttttgatgttatttataaatagaattttcttaattttattttggtttttcattgttaatatatagaaatgcaatcgatttttctatactgatcttgtatccagcaaacttgctgaacccatttattagttctaatagcttttttttttgttttttgtcgataccttgggattttctacataggagattttcacatctgagagtgaaagaagaccatttgattctttacaatttagtatgatgttagctgtaagtttctggtagtttgaggaagttaatttttgttcctggtttaagcgttttcttctttttttgtttaatcatgagtgttggagtttatccattattttatgcatctattgaagtaattgtgatttttttctttattgttgtggcatattatataaattgattttcagatgttaaaccaatcttgaattcttggaagaaatctttcttagttgtggtacaattttttatttgtttcaggattcatcttggagttttgcatctatattcataaaggatagggatgcataaaggtgtgcagttctctttttctcatgcctttgtctggcattggtatcagggtaatagtgaactcatagaatgagttcccctttcttctattttctaaaagagtttataaacaattggtattaattcttctttaaatatttgggagaatttaccagtggaagccatctaggcctgaatctttctttgtgggaagtttttatttactaattcaatctttttacctgttataggtctatttagattttctatttcttgagttagtttcaataatttgtgtctttctagggatttgtccatatcatatagtttatttaatttgttagcaatagaggttttttttttttacgttttatcccccttgaattctttttatctgtaaagttagtagtcaagtttcttctttcttgcctgatgtgagtaatttgagtcctccttcttttttgctaaagtttcgctaaagatttgtcaattttgttcaagaaccaactgttgctttatgtattttattttttatttcatttatttctactgaaattttattattttctcctttttgcttgctttcagtttcatttgttcttttatagtttcataaattgaaaggttagattattagagatattttttaaagaaataagcatttattgctataaatttagctctaatgctgctttaacttcctcccatggttttttttgtatgctgtatttttattttcattcatctcaagtatcttctaattttccttgtgatatttttttcccttgacctattggttatttatgaacgtgttgcttaatttccacatatttgtgtattccccacatttcttttagttattgatttctaaatctgtgggcatagagcctaatttacatgatttcagtcttttattatctattgtggcttattttatggcctagcacatcatatatttctgtggaatgttccgtatgcacttcagaagaatgtattttctgctgttgttgggtggagttttctatagatgtgtgttgattctacttggtttacaatgtttttcaagtctctgtatcccagttggttttctgcccagtttttctctttattgttggaagtgaggtattccagtcctcaactattattgttgaattgtctatctttcccttcaattttgtcagttgttgctttacgtattttgggattttgttattaggtacatacatacttgttattcttgttacatcttccttattgaataaattgtcatcacttaaaatgtccctcttcatctctaataagtttttgtcttacagactattttatctagtattagtatagctgccccaactctgtatgattgctgttttcatggtatatctttttctatccttttacttttcttttaaaataattttaaaaattaatttacatacactaaaatgcagagattttaagtgctcagttcaatgactgttgacaattatacacagctatgtatccacccccaaacaagatataaaccatatataatatttcatacagttttctcatgcccctttccagtcaatccccatctccttcctgtaacaggcaagtgctttctgatcataatgatctttttaaaatcatagtatattcatttgtctgttctaggttttatggtaatgaaaccaaacaggaggtattcttttgtgtctggctgctttctttccatattatgtttttaagattcatttatattgttgcatttactttttattgctgagtaatagcaaatgaatataacctagtgcagtccaaggtcagccctcttcagaaggactctgcaaaggttcactccactttccagatgataaaattgagaaaccttcaggagcattaattcttttgttactgcctctgaattaacatgtgagagaagctctcagagcttggaggaggatgactacatgatgagtttggagccaaaccctctgctccttacctcacgtatcttcctagtcatatacctaatatctggtttagtgtaaaaaatgaagaattaagaggcagaaaatacactaccctgttctacttccatcactagttcaacatatgtcatccactttctggatttttttctcctttgagtaatgaagagcttgatttggtcatctctaggatgcctttcatctctgatatactatttagttgttggtcaatgacatctaagtatgaattcgtttatgaaacacaaaagcaattttaactatgcttctctgcaatggtaaccattctcccaagagaaaggcaacaaaaagtgaagtgattcaggaatcctaattttgcccaccccacagttacacacagcacttggcctcacttattaaggaaaacagaaaacaaaaaacaaaaagtctccccattagcagggcaggaaggatacagtcccttaggaaaccaagaaaccaaatgacctgacaaatgaattaagattgtcaatgtctgctgcaccttttaggtttggaagttacaaagtaaagagtttagactaaactagaagaggatcaaatttaaggatacatgtatgtaaaagtagcatggaaagcaccagatatgactggctgtgatacaagttctggtctgcacttccacgtacaagatgtccatgcttgccttgatctcttattcccttttgagccatagtttcatctttgaaaatatttggaaatgatttattctttcttggataaagtatagaagctagttaatggcagagctgagattagaatccaggtctccttattctctgggcagtgactttcttccacatccatctttcttccttactttcacatctggtgccttacagatcctcagcacagccaagaactatacccattaggatagaagtgggaggagtagatggatttgcaggggagggttttgcagcatcctcaaacttctctcggagctggtaggctccaaagagattgagacttcgaggacagttggccattctcaaattaaacatagtacccacattcatgtgtggaaatgttcaatatttcttaggctttgaacttgataacgtagtggactatcagccctttttaatatttcttaatcactggttaatgtgaattctcagaactgagaggttcttcttgtgtagctgatttccgctgagttccttcttttttctaattttggtatgatggcactgtgtctaatgaagcaagtcaaataaacggcagattctgttccccgaagccctcttcatcctggaacattaactgtctaatttgttcatgggaagacccagctgttagcaggcagcctgcgggccccaaagcaaatgaggagaagccttcctgtgaacttcagaacacatgctggggtgggggctgtggggagacattttgtttatcactcatttaaagtatgttgctcccaaataaatggctgtaaatggagatgaagggataagacttgtgactaatttctctggggagcctaagtatctccactcctgaccccagtgtgctgcctcccccatcttcccattgtaagactcacagcagctttatgacaaggtgggtgtttatgatccagttcaggatggggactaacccagtcctccctggtggaggcattctttccatgacggggctgacgctctgccaataggatcccagtgagctcagggaacagtgtcaggttgattcagctgaggaagtcacggccttgatttagccttaaaaggctgaggttccggtggaagcgagtctgtctcagcgtgaaagcccaaggctctgagcattcccagatgacatctgtgatttttccaacacacatttggcctccttggttccttgcagtgctttggttgtgcaatcaccacttggcaggttcttcgtccagtgaaatctgtacattttcagctctgacatctcaaaaataatcattggagcattttttttatcagagtggtttatcgtaaaacaaccactcccaccgacatttcttgtaaccagtgctaggagagtgacgacttagaaggccttttgaggaaggagtagtggaagaagggctggtttcggaattgaacacaccagggttccaattctagcttccttttattacatgttgccggaccttaggccttcaggggctcagtttcatcttctataaagtagagaaaatagtatataccttgcaatgtagttgtgaggattagatatcaaatctatcattagattagttcatcagatggactcagtacactttgtatgaatatatgagtgggatgtgtgtgtgttgtgtagtgttggtcctaggttagaggtgagagtggttataagtttagtgtatatagagggaatatcagctctctttttagccctcaataaatcacaaacatgcacatacacactgcacgtgtgcacacattcttgaaaacctcagcttttttctttttgatgttgagatagctaaagattcctttctttagattttttttta

SEQ ID NO: 9072 - RNA, 9151 nt, Homo sapiens
  source 1..9151: mol_type = other RNA
actggacttggagtcagaaggccagggtttgagtcttggctctgtcatctgttgagctgggaaaatcagaataagtgcaataggcagagtcacagaggaaggactggttaatttggcctgggatggtcagggaaagcattagaggggtgagaacattttagctagttctcaaagaatgattgggagtttgtcaggtgagtgaggtgagataggggatgtgatgtattctagataaattgaatagtaacaaaaatcatatataatgaaaatgtacaacatcttcagggggtagtgagttacctgggaaggccagagctccagtgtatgggaaaactgttcaggatattgttgaaatcaggttgtgaaggcccttgaatactttttgaaggggtttggacttcaatctgctgccagaggtgctccaacttcagtttttaatcagatgggtcaaaaagtcagattcatattttacatgctgctggcagcagctctgagatgacttggagggagtgggcccagaagggagagaggaagacagaggattttttcctagtgcaggtgtgagatgagacactattgtttttcctgtctattttaataaagagtcattcatacttctgctgcagggcaagtttagtgagcatgcatggacaggtaggagtaagagactgtcctagatggtaggtgacaactggctggttatctggctgtgtcatgggtacctgagaagttccaggggagcaggctggagaggcacccctgggggtttctggtacaaggtttcaaaggcctcagtgatgagggcccagacatctttctaaggccgggatgccggccccttgggggagtcccttgatccagatagcatgacagagcactcagttttctgtgtgtgtgggcctttgaacctcttcaaagtcaagaggattttctctctgccacagacagaatattagtcctcatttatgtgcttttgtcattagaatacacgaagtatctattcttgtaaaaacctcagttgcacttggctggaagccactgttgttacatttgttggacacagctggtactctatcaagcctgaagaataaaactagtgataatcatgattccaatcagagttaattgatggagaaataatattattctatgtaacattaaaggaaaagaccactggtctggccatgtgatatggtagtgaagtgggtatttgttgtagggttatgtagaggttgaatggtgtcactagggagagtgaaaggtctcttgtggtaactagatgggaaaaggaacaaagccaatatgaacccccacaaatttatgactttgtatttacatgagaacaaaaaagactaagtagaaggaatacggggccaactggaaatgctcctgtcctacagttgttattgacttgagtgagtcacccaagcttttgtgcttgagatatcacatctgccatttaaggggaatagtttctattacttctctactgaaaaaaatacatgaagtgtcattccaatgctttcagtggtaaggattagaaatactatcaaaaataggcatccatgccaatccagccagtgagagagcactgttaacttctgtaagtaagaatagtcttgatctgtgaagtgggattagtacttacctttctggattgtcatgaaggtaaagtgtgatgagattcgcaaagtgaccagcacacctggcatctatctatatctgtagcagtatatctaatgtgtgtgtgtacacacacaagtataatagttggatgcttttattcccactccaattacatgctttcttcagtgagcccagttccaattcatatgcgggtacttgctgttttcatacccacatgttaacactgacattgacctgttctctttgaattgcaagaactggaaccaggtaggaatgtcatgggctgagtagaaagctatacgagttacaatggaaattactttgagcttacacgtcctataatcccagattaaccatatcttccaatttggagagtaattccaatataaatcactgttatggagtgctaggttgtggattactacccttttggaattaaacctaaaggcaggaattctttaggttatctctggaaactaacttcccattataaggcctagactctctactcagggcttgccagtcaatggttccccttgcctacaggttaaagtccaaagtccttggcatgacatataaggctatacatggcaagatcccagctttcctgccaccctcagctatcattaattttatcttcacatccagtactgcagccatatcagaccacttacaatttctcaaacgtcttaggtaattttaatctctgcagatgcttggaatgttctcccaccctctactggccttaccttcctacccaatctacctcatatgttaccacatcagagcatgagtccacctcatctgaatggtaactctctctcttatgcctccagtatagcttgtacatacgtccttcatagcagttacctcactgattttaatcatttgcatatttatttttctctgagttatgagctcttggaggacagagaccatatctgtagaaattggcttcatatcacctgattattcttttagaattaagtgtcatgaaataaaagctttctttgtatcttactgtattgcccacccctttcctattttcttggcaccagaaaactcagaacaaaatttaactgtagcgtacaggaattgatgatacatatcttgacattgcagtctttctagaccttttttgtctcaattttatattatctatgaatatttccaacttttattgtatatattcaggtagtcatcttcaagtcatttgaagagtgacttgtagattacactaaaaatgtcatctgatctttcaagtttccttgaaccttttcaaggtacggagcatctggcactctgccctggtttctttgtgattttgatttgcatttccctgatagctattgatattgacatttttcacgtgcttattggttggccattcatatgtcttctttggagaaatttctatttaaatcatttgctcatggaaaaaaatgggctgtttgtctttattgagttgtaagagttctgtatatattttgggtgtaagtatcttactaaatatgcaattttcaaaatttttctctcagtctgtagggttatctttttactttcttaaaaatatcccttgaagcagaaaagtttttgattttgatgaagtccaacctagccatcttttatcacctgtgctttaggtgtctaatttgaagagtcattccctaatccgagatcatgaagattgaattttgtagttgttttgaaaagagttttgtaatttagctcttacatttagatctataatacactttgagttaatttgtgtctattgtgaagtcagggtgcaaattcattcttttgcatgtgatattcagttgtccagcactatttgttaaagattattctttgcccactgaattgtcttgcctatttactgaaaatcgattgaacataaatgtgaggatttactggactcttaattctattctgttgattaatatgtttatccctataccagtaccacaccattatgattactgtcgctttgtagtatgttctggaattgggaagtgtgaatccatcaactttgttattctttttcaagattgttatagtgattctggatcccttgcatttttatatacatgttagggtcaccttgtgaatttctgtaaaaacaccagaagagttttgttaagaattgcattaagtttgtacattaatatgggaagtattgccatcttaacgatattaaatcctccaattcataagcatggtgtatctttccatttattttaatcttcagtatcactcaacagtgttttgtagtttttagcatatacattttatacttaaattgttaaatctattcctaaaaattttattccttttgatgttatttataaatagaattttcttaattttattttggtttttcattgttaatatatagaaatgcaatcgatttttctatactgatcttgtatccagcaaacttgctgaacccatttattagttctaatagcttttttttttgttttttgtcgataccttgggattttctacataggagattttcacatctgagagtgaaagaagaccatttgattctttacaatttagtatgatgttagctgtaagtttctggtagtttgaggaagttaatttttgttcctggtttaagcgttttcttctttttttgtttaatcatgagtgttggagtttatccattattttatgcatctattgaagtaattgtgatttttttctttattgttgtggcatattatataaattgattttcagatgttaaaccaatcttgaattcttggaagaaatctttcttagttgtggtacaattttttatttgtttcaggattcatcttggagttttgcatctatattcataaaggatagggatgcataaaggtgtgcagttctctttttctcatgcctttgtctggcattggtatcagggtaatagtgaactcatagaatgagttcccctttcttctattttctaaaagagtttataaacaattggtattaattcttctttaaatatttgggagaatttaccagtggaagccatctaggcctgaatctttctttgtgggaagtttttatttactaattcaatctttttacctgttataggtctatttagattttctatttcttgagttagtttcaataatttgtgtctttctagggatttgtccatatcatatagtttatttaatttgttagcaatagaggttttttttttttacgttttatcccccttgaattctttttatctgtaaagttagtagtcaagtttcttctttcttgcctgatgtgagtaatttgagtcctccttcttttttgctaaagtttcgctaaagatttgtcaattttgttcaagaaccaactgttgctttatgtattttattttttatttcatttatttctactgaaattttattattttctcctttttgcttgctttcagtttcatttgttcttttatagtttcataaattgaaaggttagattattagagatattttttaaagaaataagcatttattgctataaatttagctctaatgctgctttaacttcctcccatggttttttttgtatgctgtatttttattttcattcatctcaagtatcttctaattttccttgtgatatttttttcccttgacctattggttatttatgaacgtgttgcttaatttccacatatttgtgtattccccacatttcttttagttattgatttctaaatctgtgggcatagagcctaatttacatgatttcagtcttttattatctattgtggcttattttatggcctagcacatcatatatttctgtggaatgttccgtatgcacttcagaagaatgtattttctgctgttgttgggtggagttttctatagatgtgtgttgattctacttggtttacaatgtttttcaagtctctgtatcccagttggttttctgcccagtttttctctttattgttggaagtgaggtattccagtcctcaactattattgttgaattgtctatctttcccttcaattttgtcagttgttgctttacgtattttgggattttgttattaggtacatacatacttgttattcttgttacatcttccttattgaataaattgtcatcacttaaaatgtccctcttcatctctaataagtttttgtcttacagactattttatctagtattagtatagctgccccaactctgtatgattgctgttttcatggtatatctttttctatccttttacttttcttttaaaataattttaaaaattaatttacatacactaaaatgcagagattttaagtgctcagttcaatgactgttgacaattatacacagctatgtatccacccccaaacaagatataaaccatatataatatttcatacagttttctcatgcccctttccagtcaatccccatctccttcctgtaacaggcaagtgctttctgatcataatgatctttttaaaatcatagtatattcatttgtctgttctaggttttatggtaatgaaaccaaacaggaggtattcttttgtgtctggctgctttctttccatattatgtttttaagattcatttatattgttgcatttactttttattgctgagtaatagcaaatgaatataacctagtgcagtccaaggtcagccctcttcagaaggactctgcaaaggttcactccactttccagatgataaaattgagaaaccttcaggagcattaattcttttgttactgcctctgaattaacatgtgagagaagctctcagagcttggaggaggatgactacatgatgagtttggagccaaaccctctgctccttacctcacgtatcttcctagtcatatacctaatatctggtttagtgtaaaaaatgaagaattaagaggcagaaaatacactaccctgttctacttccatcactagttcaacatatgtcatccactttctggatttttttctcctttgagtaatgaagagcttgatttggtcatctctaggatgcctttcatctctgatatactatttagttgttggtcaatgacatctaagtatgaattcgtttatgaaacacaaaagcaattttaactatgcttctctgcaatggtaaccattctcccaagagaaaggcaacaaaaagtgaagtgattcaggaatcctaattttgcccaccccacagttacacacagcacttggcctcacttattaaggaaaacagaaaacaaaaaacaaaaagtctccccattagcagggcaggaaggatacagtcccttaggaaaccaagaaaccaaatgacctgacaaatgaattaagattgtcaatgtctgctgcaccttttaggtttggaagttacaaagtaaagagtttagactaaactagaagaggatcaaatttaaggatacatgtatgtaaaagtagcatggaaagcaccagatatgactggctgtgatacaagttctggtctgcacttccacgtacaagatgtccatgcttgccttgatctcttattcccttttgagccatagtttcatctttgaaaatatttggaaatgatttattctttcttggataaagtatagacaagaaggaagagcattgcttgaatggaagcatgtcccagacactttatcactggtgaagagccgagctcattgtctaaacttggctcctcattttaaaaagtaaaaaaacgagttatcaaaatgattagttattcttgagtctcacagctagttaatggcagagctgagattagaatccaggtctccttattctctgggcagtgactttcttccacatccatctttcttccttactttcacatctggtgccttacagatcctcagcacagccaagaactatacccattaggatagaagtgggaggagtagatggatttgcaggggagggttttgcagcatcctcaaacttctctcggagctggtaggctccaaagagattgagacttcgaggacagttggccattctcaaattaaacatagtacccacattcatgtgtggaaatgttcaatatttcttaggctttgaacttgataacgtagtggactatcagccctttttaatatttcttaatcactggttaatgtgaattctcagaactgagaggttcttcttgtgtagctgatttccgctgagttccttcttttttctaattttggtatgatggcactgtgtctaatgaagcaagtcaaataaacggcagattctgttccccgaagccctcttcatcctggaacattaactgtctaatttgttcatgggaagacccagctgttagcaggcagcctgcgggccccaaagcaaatgaggagaagccttcctgtgaacttcagaacacatgctggggtgggggctgtggggagacattttgtttatcactcatttaaagtatgttgctcccaaataaatggctgtaaatggagatgaagggataagacttgtgactaatttctctggggagcctaagtatctccactcctgaccccagtgtgctgcctcccccatcttcccattgtaagactcacagcagctttatgacaaggtgggtgtttatgatccagttcaggatggggactaacccagtcctccctggtggaggcattctttccatgacggggctgacgctctgccaataggatcccagtgagctcagggaacagtgtcaggttgattcagctgaggaagtcacggccttgatttagccttaaaaggctgaggttccggtggaagcgagtctgtctcagcgtgaaagcccaaggctctgagcattcccagatgacatctgtgatttttccaacacacatttggcctccttggttccttgcagtgctttggttgtgcaatcaccacttggcaggttcttcgtccagtgaaatctgtacattttcagctctgacatctcaaaaataatcattggagcattttttttatcagagtggtttatcgtaaaacaaccactcccaccgacatttcttgtaaccagtgctaggagagtgacgacttagaaggccttttgaggaaggagtagtggaagaagggctggtttcggaattgaacacaccagggttccaattctagcttccttttattacatgttgccggaccttaggccttcaggggctcagtttcatcttctataaagtagagaaaatagtatataccttgcaatgtagttgtgaggattagatatcaaatctatcattagattagttcatcagatggactcagtacactttgtatgaatatatgagtgggatgtgtgtgtgttgtgtagtgttggtcctaggttagaggtgagagtggttataagtttagtgtatatagagggaatatcagctctctttttagccctcaataaatcacaaacatgcacatacacactgcacgtgtgcacacattcttgaaaacctcagcttttttctttttgatgttgagatagctaaagattcctttctttagattttttttta

SEQ ID NO: 9073 - RNA, 2405 nt, Homo sapiens
  source 1..2405: mol_type = other RNA
actggacttggagtcagaaggccattgtcgatagaaaataattcagggtgcaatgtgatgcctttgacctgttcaaatggtttcagaccagaatccttcccaagtctcaccatatcttcgaggatagcttttttgacatccttatttctgcacagttcctcaaacgacccttcaaatcctctcttttgggcccaggaacataatgtctcaacatctggtaccacaattgcaatgagaaatgcctgcaggctttctccgtggacaaacacctgagcaacaggctcacttcgcatgtagatattttcaatcttttcaggggctatgtattctccttgtgccagcttaaatatgtgctttttccggtcgataattttcaaggtgccatttggtaaccattttccaatgtcccctgtgtgtaaccagccgtctttgtccaaagcttctgctgttttcgctgggtccttcaagtagccctgaaatacatttggccctttcacacacacctcgccctcgccctcggcagccatgtaattcatttcttccacatcaacaagttttatcaaattgcacggcatcggggccccaacatggcctgcggtccagtctccaggcatggtcaggcagcacccggcagtgcactctgtctgtccgtatccttcataaaactgacagcccagggctgctctgaggaacgtcagcacagtggcagacaccggggcggctcctgtcaccatcagccggactcttccgcccaggctcgactgtactttgtggaagatcagccggtcccacaggctgttgtttctgatgatgccgctgcgaagctctgcttctttcctcttggaggcaaagtccaagagccatcgcttcagcgtggtgtttgcttgtccgaaaattcggtcaaacatccggttcagcagtcttggaaccacggggaagacagtgggttgaagcaccttgaggtcatccatgagcagcctgatatctccttggaaaaatccgattttagctccatgacacagcattacacactctacaactctctcaaacatatgggcgagaggcaagaaagatatcaaagtatcatctgggcaaggattgactgtattctctgttgctttcacaaaagctgaacaatcgctcactatgtttcggtgagtgaccattgctcctttggggttgcctgtagttccacttgtgaaacaaattactgcaagatcttcaggtgctggaggcttgggcttccgtctgttggctcttcccaggtcctccatcgccttcatgctggtgacttccaccccacacctctggcctcgttccaccagttcactgccgtaggcatccatgacaactatgattttaaggcctggtattaacttattttctacaccctctaataagagtttggccttctctggcttgtcaacaaaaaccagagagagttcagctttgttgactatgtacgtgatggcttcatttccaagggtatcataaagtggaacgatcaccatcgaataagcaaagcatccttgttcaataatcacccactcaggtctattttgagcaaagatgccaatgaactgatctggggcagtcttgaagcccttctggatcagtgctgagcctatgcactccgacaattctgcaacctgtttatatgaaagccattcatagggttggtctggtttccgagagcctaaacaagggccattatatatttgaccatggagcccccagggccacagggaacatctagagggtccagtgagctttgggaccgactctgggaaagttacagtggacacagaggggcctgagcgatcttgacacctgtattcccctctggaaaccttcgtataatgttgtgacatcatcatagaaatacaccaagggctcgtcgctgtcaagtagtgcggatcttcgtgcaccaccactacccgccacttccactgactgcatggagaggtcgcatggcggcttcaggggtttgggtctcgtggcgtaccagaaggtggtgagtgctgcaaaagctccgaagcccataagcgtgttggtcggaagagtacgcacgtactgtcggaagtcaaccagctctggcattcgaaaataccggaacagctcatgggcttgcattgtcctgtgttgatagttctctaagctgaattattaacattgtattctcttcatgtcatttagaaaccaaaaaccgggtggtctggatgtttctctccttctaaagttcctcaagctttcatcaagatgaataatggcagtttgatggaatacttcactaggaatgcagccctcaaacaaacccacataaatgacacccttgcccctgcagtggcaaattaagaaagcctgacatctttccttaacgcagcaacccaagctggcaagatgct

SEQ ID NO: 9074 - RNA, 2279 nt, Homo sapiens
  source 1..2279: mol_type = other RNA
actggacttggagtcagaaggccattgtcgatagaaaataattcagggtgcaatgtgatgcctttgacctgttcaaatggtttcagaccagaatccttcccaagtctcaccatatcttcgaggatagcttttttgacatccttatttctgcacagttcctcaaacgacccttcaaatcctctcttttgggcccaggaacataatgtctcaacatctggtaccacaattgcaatgagaaatgcctgcaggctttctccgtggacaaacacctgagcaacaggctcacttcgcatgtagatattttcaatcttttcaggggctatgtattctccttgtgccagcttaaatatgtgctttttccggtcgataattttcaaggtgccatttggtaaccattttccaatgtcccctgtgtgtaaccagccgtctttgtccaaagcttctgctgttttcgctgggtccttcaagtagccctgaaatacatttggccctttcacacacacctcgccctcgccctcggcagccatgtaattcatttcttccacatcaacaagttttatcaaattgcacggcatcggggccccaacatggcctgcggtccagtctccaggcatggtcaggcagcacccggcagtgcactctgtctgtccgtatccttcataaaactgacagcccagggctgctctgaggaacgtcagcacagtggcagacaccggggcggctcctgtcaccatcagccggactcttccgcccaggctcgactgtactttgtggaagatcagccggtcccacaggctgttgtttctgatgatgccgctgcgaagctctgcttctttcctcttggaggcaaagtccaagagccatcgcttcagcgtggtgtttgcttgtccgaaaattcggtcaaacatccggttcagcagtcttggaaccacggggaagacagtgggttgaagcaccttgaggtcatccatgagcagcctgatatctccttggaaaaatccgattttagctccatgacacagcattacacactctacaactctctcaaacatatgggcgagaggcaagaaagatatcaaagtatcatctgggcaaggattgactgtattctctgttgctttcacaaaagctgaacaatcgctcactatgtttcggtgagtgaccattgctcctttggggttgcctgtagttccacttgtgaaacaaattactgcaagatcttcaggtgctggaggcttgggcttccgtctgttggctcttcccaggtcctccatcgccttcatgctggtgacttccaccccacacctctggcctcgttccaccagttcactgccgtaggcatccatgacaactatgattttaaggcctggtattaacttattttctacaccctctaataagagtttggccttctctggcttgtcaacaaaaaccagagagagttcagctttgttgactatgtacgtgatggcttcatttccaagggtatcataaagtggaacgatcaccatcgaataagcaaagcatccttgttcaataatcacccactcaggtctattttgagcaaagatgccaatgaactgatctggggcagtcttgaagcccttctggatcagtgctgagcctatgcactccgacaattctgcaacctgtttatatgaaagccattcatagggttggtctggtttccgagagcctaaacaagggccattatatatttgaccatggagcccccagggccacagggaacatctagagggtccagtgagctttgggaccgactctgggaaagttacagtggacacagaggggcctgagcgatcttgacacctgtattcccctctggaaaccttcgtataatgttgtgacatcatcatagaaatacaccaagggctcgtcgctgtcaagtagtgcggatcttcgtgcaccaccactacccgccacttccactgactgcatggagaggtcgcatggcggcttcaggggtttgggtctcgtggcgtaccagaaggtggtgagtgctgcaaaagctccgaagcccataagcgtgttggtcggaagagtacgcacgtactgtcggaagtcaaccagctctggcattcgaaaataccggaacagctcatgggcttgcattgtcctgtgttgatagttctctaagctgaattcatgacagcaaagaaagaacagataagcagatttcttcaggccatggttctggaaagaaggcaccagcacttaacaaaaccactcaccatctgtgccaccaacagctgactact

SEQ ID NO: 9075 - RNA, 2431 nt, Homo sapiens
  source 1..2431: mol_type = other RNA
actggacttggagtcagaaggccattgtcgatagaaaataattcagggtgcaatgtgatgcctttgacctgttcaaatggtttcagaccagaatccttcccaagtctcaccatatcttcgaggatagcttttttgacatccttatttctgcacagttcctcaaacgacccttcaaatcctctcttttgggcccaggaacataatgtctcaacatctggtaccacaattgcaatgagaaatgcctgcaggctttctccgtggacaaacacctgagcaacaggctcacttcgcatgtagatattttcaatcttttcaggggctatgtattctccttgtgccagcttaaatatgtgctttttccggtcgataattttcaaggtgccatttggtaaccattttccaatgtcccctgtgtgtaaccagccgtctttgtccaaagcttctgctgttttcgctgggtccttcaagtagccctgaaatacatttggccctttcacacacacctcgccctcgccctcggcagccatgtaattcatttcttccacatcaacaagttttatcaaattgcacggcatcggggccccaacatggcctgcggtccagtctccaggcatggtcaggcagcacccggcagtgcactctgtctgtccgtatccttcataaaactgacagcccagggctgctctgaggaacgtcagcacagtggcagacaccggggcggctcctgtcaccatcagccggactcttccgcccaggctcgactgtactttgtggaagatcagccggtcccacaggctgttgtttctgatgatgccgctgcgaagctctgcttctttcctcttggaggcaaagtccaagagccatcgcttcagcgtggtgtttgcttgtccgaaaattcggtcaaacatccggttcagcagtcttggaaccacggggaagacagtgggttgaagcaccttgaggtcatccatgagcagcctgatatctccttggaaaaatccgattttagctccatgacacagcattacacactctacaactctctcaaacatatgggcgagaggcaagaaagatatcaaagtatcatctgggcaaggattgactgtattctctgttgctttcacaaaagctgaacaatcgctcactatgtttcggtgagtgaccattgctcctttggggttgcctgtagttccacttgtgaaacaaattactgcaagatcttcaggtgctggaggcttgggcttccgtctgttggctcttcccaggtcctccatcgccttcatgctggtgacttccaccccacacctctggcctcgttccaccagttcactgccgtaggcatccatgacaactatgattttaaggcctggtattaacttattttctacaccctctaataagagtttggccttctctggcttgtcaacaaaaaccagagagagttcagctttgttgactatgtacgtgatggcttcatttccaagggtatcataaagtggaacgatcaccatcgaataagcaaagcatccttgttcaataatcacccactcaggtctattttgagcaaagatgccaatgaactgatctggggcagtcttgaagcccttctggatcagtgctgagcctatgcactccgacaattctgcaacctgtttatatgaaagccattcatagggttggtctggtttccgagagcctaaacaagggccattatcataaaatacaggatgtgacactcacatatttgaccatggagcccccagggccacagggaacatctagagggtccagtgagctttgggaccgactctgggaaagttacagtggacacagaggggcctgagcgatcttgacacctgtattcccctctggaaaccttcgtataatgttgtgacatcatcatagaaatacaccaagggctcgtcgctgtcaagtagtgcggatcttcgtgcaccaccactacccgccacttccactgactgcatggagaggtcgcatggcggcttcaggggtttgggtctcgtggcgtaccagaaggtggtgagtgctgcaaaagctccgaagcccataagcgtgttggtcggaagagtacgcacgtactgtcggaagtcaaccagctctggcattcgaaaataccggaacagctcatgggcttgcattgtcctgtgttgatagttctctaagctgaattattaacattgtattctcttcatgtcatttagaaaccaaaaaccgggtggtctggatgtttctctccttctaaagttcctcaagctttcatcaagatgaataatggcagtttgatggaatacttcactaggaatgcagccctcaaacaaacccacataaatgacacccttgcccctgcagtggcaaattaagaaagcctgacatctttccttaacgcagcaacccaagctggcaagatgct

SEQ ID NO: 9076 - RNA, 1943 nt, Homo sapiens
  source 1..1943: mol_type = other RNA
actggacttggagtcagaaggccattgtcgatagaaaataattcagggtgcaatgtgatgcctttgacctgttcaaatggtttcagaccagaatccttcccaagtctcaccatatcttcgaggatagcttttttgacatccttatttctgcacagttcctcaaacgacccttcaaatcctctcttttgggcccaggaacataatgtctcaacatctggtaccacaattgcaatgagaaatgcctgcaggctttctccgtggacaaacacctgagcaacaggctcacttcgcatgtagatattttcaatcttttcaggggctatgtattctccttgtgccagcttaaatatgtgctttttccggtcgataattttcaaggtgccatttggtaaccattttccaatgtcccctgtgtgtaaccagccgtctttgtccaaagcttctgctgttttcgctgggtccttcaagtagccctgaaatacatttggccctttcacacacacctcgccctcgccctcggcagccatgtaattcatttcttccacatcaacaagttttatcaaattgcacggcatcggggccccaacatggcctgcggtccagtctccaggcatggtcaggcagcacccggcagtgcactctgtctgtccgtatccttcataaaactgacagcccagggctgctctgaggaacgtcagcacagtggcagacaccggggcggctcctgtcaccatcagccggactcttccgcccaggctcgactgtactttgtggaagatcagccggtcccacaggctgttgtttctgatgatgccgctgcgaagctctgcttctttcctcttggaggcaaagtccaagagccatcgcttcagcgtggtgtttgcttgtccgaaaattcggtcaaacatccggttcagcagtcttggaaccacggggaagacagtgggttgaagcaccttgaggtcatccatgagcagcctgatatctccttggaaaaatccgattttagctccatgacacagcattacacactctacaactctctcaaacatatgggcgagaggcaagaaagatatcaaagtatcatctgggcaaggattgactgtattctctgttgctttcacaaaagctgaacaatcgctcactatgtttcggtgagtgaccattgctcctttggggttgcctgtagttccacttgtgaaacaaattactgcaagatcttcaggtgctggaggcttgggcttccgtctgttggctcttcccaggtcctccatcgccttcatgctggtgacttccaccccacacctctggcctcgttccaccagttcactgccgtaggcatccatgacaactatgattttaaggcctggtattaacttattttctacaccctctaataagagtttggccttctctggcttgtcaacaaaaaccagagagagttcagctttgttgactatgtacgtgatggcttcatttccaagggtatcataaagtggaacgatcaccatcgaataagcaaagcatccttgttcaataatcacccactcaggtctattttgagcaaagatgccaatgaactgatctggggcagtcttgaagcccttctggatcagtgctgagcctatgcactccgacaattctgcaacctgtttatatgaaagccattcatagggttggtctggtttccgagagcctaaacaagggccattatttgacacctgtattcccctctggaaaccttcgtataatgttgtgacatcatcatagaaatacaccaagggctcgtcgctgtcaagtagtgcggatcttcgtgcaccaccactacccatgacagcaaagaaagaacagataagcagatttcttcaggccatggttctggaaagaaggcaccagcacttaacaaaaccactcaccatctgtgccaccaacagctgactact

SEQ ID NO: 9077 - RNA, 2183 nt, Homo sapiens
  source 1..2183: mol_type = other RNA
actggacttggagtcagaaggccattgtcgatagaaaataattcagggtgcaatgtgatgcctttgacctgttcaaatggtttcagaccagaatccttcccaagtctcaccatatcttcgaggatagcttttttgacatccttatttctgcacagttcctcaaacgacccttcaaatcctctcttttgggcccaggaacataatgtctcaacatctggtaccacaattgcaatgagaaatgcctgcaggctttctccgtggacaaacacctgagcaacaggctcacttcgcatgtagatattttcaatcttttcaggggctatgtattctccttgtgccagcttaaatatgtgctttttccggtcgataattttcaaggtgccatttggtaaccattttccaatgtcccctgtgtgtaaccagccgtctttgtccaaagcttctgctgttttcgctgggtccttcaagtagccctgaaatacatttggccctttcacacacacctcgccctcgccctcggcagccatgtaattcatttcttccacatcaacaagttttatcaaattgcacggcatcggggccccaacatggcctgcggtccagtctccaggcatggtcaggcagcacccggcagtgcactctgtctgtccgtatccttcataaaactgacagcccagggctgctctgaggaacgtcagcacagtggcagacaccggggcggctcctgtcaccatcagccggactcttccgcccaggctcgactgtactttgtggaagatcagccggtcccacaggctgttgtttctgatgatgccgctgcgaagctctgcttctttcctcttggaggcaaagtccaagagccatcgcttcagcgtggtgtttgcttgtccgaaaattcggtcaaacatccggttcagcagtcttggaaccacggggaagacagtgggttgaagcaccttgaggtcatccatgagcagcctgatatctccttggaaaaatccgattttagctccatgacacagcattacacactctacaactctctcaaacatatgggcgagaggcaagaaagatatcaaagtatcatctgggcaaggattgactgtattctctgttgctttcacaaaagctgaacaatcgctcactatgtttcggtgagtgaccattgctcctttggggttgcctgtagttccacttgtgaaacaaattactgcaagatcttcaggtgctggaggcttgggcttccgtctgttggctcttcccaggtcctccatcgccttcatgctggtgacttccaccccacacctctggcctcgttccaccagttcactgccgtaggcatccatgacaactatgattttaaggcctggtattaacttattttctacaccctctaataagagtttggccttctctggcttgtcaacaaaaaccagagagagttcagctttgttgactatgtacgtgatggcttcatttccaagggtatcataaagtggaacgatcaccatcgaataagcaaagcatccttgttcaataatcacccactcaggtctattttgagcaaagatgccaatgaactgatctggggcagtcttgaagcccttctggatcagtgctgagcctatgcactccgacaattctgcaacctgtttatatgaaagccattcatagggttggtctggtttccgagagcctaaacaagggccattatttgacacctgtattcccctctggaaaccttcgtataatgttgtgacatcatcatagaaatacaccaagggctcgtcgctgtcaagtagtgcggatcttcgtgcaccaccactacccgccacttccactgactgcatggagaggtcgcatggcggcttcaggggtttgggtctcgtggcgtaccagaaggtggtgagtgctgcaaaagctccgaagcccataagcgtgttggtcggaagagtacgcacgtactgtcggaagtcaaccagctctggcattcgaaaataccggaacagctcatgggcttgcattgtcctgtgttgatagttctctaagctgaattaaggttttctttgccttcagcaagtttaggatatcaatgaagacaaacacacctgcaagagttaacagagctacagaagacagatctgataaccacggcaggtagggccctggtgctccaggaatct

SEQ ID NO: 9078 - RNA, 2148 nt, Homo sapiens
  source 1..2148: mol_type = other RNA
actggacttggagtcagaaggccattgtcgatagaaaataattcagggtgcaatgtgatgcctttgacctgttcaaatggtttcagaccagaatccttcccaagtctcaccatatcttcgaggatagcttttttgacatccttatttctgcacagttcctcaaacgacccttcaaatcctctcttttgggcccaggaacataatgtctcaacatctggtaccacaattgcaatgagaaatgcctgcaggctttctccgtggacaaacacctgagcaacaggctcacttcgcatgtagatattttcaatcttttcaggggctatgtattctccttgtgccagcttaaatatgtgctttttccggtcgataattttcaaggtgccatttggtaaccattttccaatgtcccctgtgtgtaaccagccgtctttgtccaaagcttctgctgttttcgctgggtccttcaagtagccctgaaatacatttggccctttcacacacacctcgccctcgccctcggcagccatgtaattcatttcttccacatcaacaagttttatcaaattgcacggcatcggggccccaacatggcctgcggtccagtctccaggcatggtcaggcagcacccggcagtgcactctgtctgtccgtatccttcataaaactgacagcccagggctgctctgaggaacgtcagcacagtggcagacaccggggcggctcctgtcaccatcagccggactcttccgcccaggctcgactgtactttgtggaagatcagccggtcccacaggctgttgtttctgatgatgccgctgcgaagctctgcttctttcctcttggaggcaaagtccaagagccatcgcttcagcgtggtgtttgcttgtccgaaaattcggtcaaacatccggttcagcagtcttggaaccacggggaagacagtgggttgaagcaccttgaggtcatccatgagcagcctgatatctccttggaaaaatccgattttagctccatgacacagcattacacactctacaactctctcaaacatatgggcgagaggcaagaaagatatcaaagtatcatctgggcaaggattgactgtattctctgttgctttcacaaaagctgaacaatcgctcactatgtttcggtgagtgaccattgctcctttggggttgcctgtagttccacttgtgaaacaaattactgcaagatcttcaggtgctggaggcttgggcttccgtctgttggctcttcccaggtcctccatcgccttcatgctggtgacttccaccccacacctctggcctcgttccaccagttcactgccgtaggcatccatgacaactatgattttaaggcctggtattaacttattttctacaccctctaataagagtttggccttctctggcttgtcaacaaaaaccagagagagttcagctttgttgactatgtacgtgatggcttcatttccaagggtatcataaagtggaacgatcaccatcgaataagcaaagcatccttgttcaataatcacccactcaggtctattttgagcaaagatgccaatgaactgatctggggcagtcttgaagcccttctggatcagtgctgagcctatgcactccgacaattctgcaacctgtttatatgaaagccattcatagggttggtctggtttccgagagcctaaacaagggccattatttgacacctgtattcccctctggaaaccttcgtataatgttgtgacatcatcatagaaatacaccaagggctcgtcgctgtcaagtagtgcggatcttcgtgcaccaccactacccgccacttccactgactgcatggagaggtcgcatggcggcttcaggggtttgggtctcgtggcgtaccagaaggtggtgagtgctgcaaaagctccgaagcccataagcgtgttggtcggaagagtacgcacgtactgtcggaagtcaaccagctctggcattcgaaaataccggaacagctcatgggcttgcattgtcctgtgttgatagttctctaagctgaattagcgaatggtacttagtacctatgtagatgcttcttcctctccccggccagggtctcctcccatctgtctttatatgcccttggttcttaac

SEQ ID NO: 9079 - RNA, 2296 nt, Homo sapiens
  source 1..2296: mol_type = other RNA
actggacttggagtcagaaggccattgtcgatagaaaataattcagggtgcaatgtgatgcctttgacctgttcaaatggtttcagaccagaatccttcccaagtctcaccatatcttcgaggatagcttttttgacatccttatttctgcacagttcctcaaacgacccttcaaatcctctcttttgggcccaggaacataatgtctcaacatctggtaccacaattgcaatgagaaatgcctgcaggctttctccgtggacaaacacctgagcaacaggctcacttcgcatgtagatattttcaatcttttcaggggctatgtattctccttgtgccagcttaaatatgtgctttttccggtcgataattttcaaggtgccatttggtaaccattttccaatgtcccctgtgtgtaaccagccgtctttgtccaaagcttctgctgttttcgctgggtccttcaagtagccctgaaatacatttggccctttcacacacacctcgccctcgccctcggcagccatgtaattcatttcttccacatcaacaagttttatcaaattgcacggcatcggggccccaacatggcctgcggtccagtctccaggcatggtcaggcagcacccggcagtgcactctgtctgtccgtatccttcataaaactgacagcccagggctgctctgaggaacgtcagcacagtggcagacaccggggcggctcctgtcaccatcagccggactcttccgcccaggctcgactgtactttgtggaagatcagccggtcccacaggctgttgtttctgatgatgccgctgcgaagctctgcttctttcctcttggaggcaaagtccaagagccatcgcttcagcgtggtgtttgcttgtccgaaaattcggtcaaacatccggttcagcagtcttggaaccacggggaagacagtgggttgaagcaccttgaggtcatccatgagcagcctgatatctccttggaaaaatccgattttagctccatgacacagcattacacactctacaactctctcaaacatatgggcgagaggcaagaaagatatcaaagtatcatctgggcaaggattgactgtattctctgttgctttcacaaaagctgaacaatcgctcactatgtttcggtgagtgaccattgctcctttggggttgcctgtagttccacttgtgaaacaaattactgcaagatcttcaggtgctggaggcttgggcttccgtctgttggctcttcccaggtcctccatcgccttcatgctggtgacttccaccccacacctctggcctcgttccaccagttcactgccgtaggcatccatgacaactatgattttaaggcctggtattaacttattttctacaccctctaataagagtttggccttctctggcttgtcaacaaaaaccagagagagttcagctttgttgactatgtacgtgatggcttcatttccaagggtatcataaagtggaacgatcaccatcgaataagcaaagcatccttgttcaataatcacccactcaggtctattttgagcaaagatgccaatgaactgatctggggcagtcttgaagcccttctggatcagtgctgagcctatgcactccgacaattctgcaacctgtttatatgaaagccattcatagggttggtctggtttccgagagcctaaacaagggccattatttgacacctgtattcccctctggaaaccttcgtataatgttgtgacatcatcatagaaatacaccaagggctcgtcgctgtcaagtagtgcggatcttcgtgcaccaccactacccgccacttccactgactgcatggagaggtcgcatggcggcttcaggggtttgggtctcgtggcgtaccagaaggtggtgagtgctgcaaaagctccgaagcccataagcgtgttggtcggaagagtacgcacgtactgtcggaagtcaaccagctctggcattcgaaaataccggaacagctcatgggcttgcattgtcctgtgttgatagttctctaagctgaattattaacattgtattctcttcatgtcatttagaaaccaaaaaccgggtggtctggatgtttctctccttctaaagttcctcaagctttcatcaagatgaataatggcagtttgatggaatacttcactaggaatgcagccctcaaacaaacccacataaatgacacccttgcccctgcagtggcaaattaagaaagcctgacatctttccttaacgcagcaacccaagctggcaagatgct

SEQ ID NO: 9080 - RNA, 2083 nt, Homo sapiens
  source 1..2083: mol_type = other RNA
actggacttggagtcagaaggccattgtcgatagaaaataattcagggtgcaatgtgatgcctttgacctgttcaaatggtttcagaccagaatccttcccaagtctcaccatatcttcgaggatagcttttttgacatccttatttctgcacagttcctcaaacgacccttcaaatcctctcttttgggcccaggaacataatgtctcaacatctggtaccacaattgcaatgagaaatgcctgcaggctttctccgtggacaaacacctgagcaacaggctcacttcgcatgtagatattttcaatcttttcaggggctatgtattctccttgtgccagcttaaatatgtgctttttccggtcgataattttcaaggtgccatttggtaaccattttccaatgtcccctgtgtgtaaccagccgtctttgtccaaagcttctgctgttttcgctgggtccttcaagtagccctgaaatacatttggccctttcacacacacctcgccctcgccctcggcagccatgtaattcatttcttccacatcaacaagttttatcaaattgcacggcatcggggccccaacatggcctgcggtccagtctccaggcatggtcaggcagcacccggcagtgcactctgtctgtccgtatccttcataaaactgacagcccagggctgctctgaggaacgtcagcacagtggcagacaccggggcggctcctgtcaccatcagccggactcttccgcccaggctcgactgtactttgtggaagatcagccggtcccacaggctgttgtttctgatgatgccgctgcgaagctctgcttctttcctcttggaggcaaagtccaagagccatcgcttcagcgtggtgtttgcttgtccgaaaattcggtcaaacatccggttcagcagtcttggaaccacggggaagacagtgggttgaagcaccttgaggtcatccatgagcagcctgatatctccttggaaaaatccgattttagctccatgacacagcattacacactctacaactctctcaaacatatgggcgagaggcaagaaagatatcaaagtatcatctgggcaaggattgactgtattctctgttgctttcacaaaagctgaacaatcgctcactatgtttcggtgagtgaccattgctcctttggggttgcctgtagttccacttgtgaaacaaattactgcaagatcttcaggtgctggaggcttgggcttccgtctgttggctcttcccaggtcctccatcgccttcatgctggtgacttccaccccacacctctggcctcgttccaccagttcactgccgtaggcatccatgacaactatgattttaaggcctggtattaacttattttctacaccctctaataagagtttggccttctctggcttgtcaacaaaaaccagagagagttcagctttgttgactatgtacgtgatggcttcatttccaagggtatcataaagtggaacgatcaccatcgaataagcaaagcatccttgttcaataatcacccactcaggtctattttgagcaaagatgccaatgaactgatctggggcagtcttgaagcccttctggatcagtgctgagcctatgcactccgacaattctgcaacctgtttatatgaaagccattcatagggttggtctggtttccgagagcctaaacaagggccattatttgacacctgtattcccctctggaaaccttcgtataatgttgtgacatcatcatagaaatacaccaagggctcgtcgctgtcaagtagtgcggatcttcgtgcaccaccactacccgccacttccactgactgcatggagaggtcgcatggcggcttcaggggtttgggtctcgtggcgtaccagaaggtggtgagtgctgcaaaagctccgaagcccataagcgtgttggtcggaagagtacgcacgtactgtcggaagtcaaccagctctggcattcgaaaataccggaacagctcatgggcttgcattgtcctgtgttgatagttctctaagctgaattcatctgtgccaccaacagctgactact

SEQ ID NO: 9081 - RNA, 2170 nt, Homo sapiens
  source 1..2170: mol_type = other RNA
actggacttggagtcagaaggccattgtcgatagaaaataattcagggtgcaatgtgatgcctttgacctgttcaaatggtttcagaccagaatccttcccaagtctcaccatatcttcgaggatagcttttttgacatccttatttctgcacagttcctcaaacgacccttcaaatcctctcttttgggcccaggaacataatgtctcaacatctggtaccacaattgcaatgagaaatgcctgcaggctttctccgtggacaaacacctgagcaacaggctcacttcgcatgtagatattttcaatcttttcaggggctatgtattctccttgtgccagcttaaatatgtgctttttccggtcgataattttcaaggtgccatttggtaaccattttccaatgtcccctgtgtgtaaccagccgtctttgtccaaagcttctgctgttttcgctgggtccttcaagtagccctgaaatacatttggccctttcacacacacctcgccctcgccctcggcagccatgtaattcatttcttccacatcaacaagttttatcaaattgcacggcatcggggccccaacatggcctgcggtccagtctccaggcatggtcaggcagcacccggcagtgcactctgtctgtccgtatccttcataaaactgacagcccagggctgctctgaggaacgtcagcacagtggcagacaccggggcggctcctgtcaccatcagccggactcttccgcccaggctcgactgtactttgtggaagatcagccggtcccacaggctgttgtttctgatgatgccgctgcgaagctctgcttctttcctcttggaggcaaagtccaagagccatcgcttcagcgtggtgtttgcttgtccgaaaattcggtcaaacatccggttcagcagtcttggaaccacggggaagacagtgggttgaagcaccttgaggtcatccatgagcagcctgatatctccttggaaaaatccgattttagctccatgacacagcattacacactctacaactctctcaaacatatgggcgagaggcaagaaagatatcaaagtatcatctgggcaaggattgactgtattctctgttgctttcacaaaagctgaacaatcgctcactatgtttcggtgagtgaccattgctcctttggggttgcctgtagttccacttgtgaaacaaattactgcaagatcttcaggtgctggaggcttgggcttccgtctgttggctcttcccaggtcctccatcgccttcatgctggtgacttccaccccacacctctggcctcgttccaccagttcactgccgtaggcatccatgacaactatgattttaaggcctggtattaacttattttctacaccctctaataagagtttggccttctctggcttgtcaacaaaaaccagagagagttcagctttgttgactatgtacgtgatggcttcatttccaagggtatcataaagtggaacgatcaccatcgaataagcaaagcatccttgttcaataatcacccactcaggtctattttgagcaaagatgccaatgaactgatctggggcagtcttgaagcccttctggatcagtgctgagcctatgcactccgacaattctgcaacctgtttatatgaaagccattcatagggttggtctggtttccgagagcctaaacaagggccattatttgacacctgtattcccctctggaaaccttcgtataatgttgtgacatcatcatagaaatacaccaagggctcgtcgctgtcaagtagtgcggatcttcgtgcaccaccactacccgccacttccactgactgcatggagaggtcgcatggcggcttcaggggtttgggtctcgtggcgtaccagaaggtggtgagtgctgcaaaagctccgaagcccataagcgtgttggtcggaagagtacgcacgtactgtcggaagtcaaccagctctggcattcgaaaataccggaacagctcatgggcttgcattgtcctgtgttgatagttctctaagctgaattcatgacagcaaagaaagaacagataagcagatttcttcaggccatggttctggaaagaaggcaccagcacttaacaaaaccactcaccatctgtgccaccaacagctgactact

SEQ ID NO: 9082 - RNA, 2180 nt, Homo sapiens
  source 1..2180: mol_type = other RNA
actggacttggagtcagaaggccattgtcgatagaaaataattcagggtgcaatgtgatgcctttgacctgttcaaatggtttcagaccagaatccttcccaagtctcaccatatcttcgaggatagcttttttgacatccttatttctgcacagttcctcaaacgacccttcaaatcctctcttttgggcccaggaacataatgtctcaacatctggtaccacaattgcaatgagaaatgcctgcaggctttctccgtggacaaacacctgagcaacaggctcacttcgcatgtagatattttcaatcttttcaggggctatgtattctccttgtgccagcttaaatatgtgctttttccggtcgataattttcaaggtgccatttggtaaccattttccaatgtcccctgtgtgtaaccagccgtctttgtccaaagcttctgctgttttcgctgggtccttcaagtagccctgaaatacatttggccctttcacacacacctcgccctcgccctcggcagccatgtaattcatttcttccacatcaacaagttttatcaaattgcacggcatcggggccccaacatggcctgcggtccagtctccaggcatggtcaggcagcacccggcagtgcactctgtctgtccgtatccttcataaaactgacagcccagggctgctctgaggaacgtcagcacagtggcagacaccggggcggctcctgtcaccatcagccggactcttccgcccaggctcgactgtactttgtggaagatcagccggtcccacaggctgttgtttctgatgatgccgctgcgaagctctgcttctttcctcttggaggcaaagtccaagagccatcgcttcagcgtggtgtttgcttgtccgaaaattcggtcaaacatccggttcagcagtcttggaaccacggggaagacagtgggttgaagcaccttgaggtcatccatgagcagcctgatatctccttggaaaaatccgattttagctccatgacacagcattacacactctacaactctctcaaacatatgggcgagaggcaagaaagatatcaaagtatcatctgggcaaggattgactgtattctctgttgctttcacaaaagctgaacaatcgctcactatgtttcggtgagtgaccattgctcctttggggttgcctgtagttccacttgtgaaacaaattactgcaagatcttcaggtgctggaggcttgggcttccgtctgttggctcttcccaggtcctccatcgccttcatgctggtgacttccaccccacacctctggcctcgttccaccagttcactgccgtaggcatccatgacaactatgattttaaggcctggtattaacttattttctacaccctctaataagagtttggccttctctggcttgtcaacaaaaaccagagagagttcagctttgttgactatgtacgtgatggcttcatttccaagggtatcataaagtggaacgatcaccatcgaataagcaaagcatccttgttcaataatcacccactcaggtctattttgagcaaagatgccaatgaactgatctggggcagtcttgaagcccttctggatcagtgctgagcctatgcactccgacaattctgcaacctgtttatatgaaagccattcatagggttggtctggtttccgagagcctaaacaagggccattatttgacacctgtattcccctctggaaaccttcgtataatgttgtgacatcatcatagaaatacaccaagggctcgtcgctgtcaagtagtgcggatcttcgtgcaccaccactacccgccacttccactgactgcatggagaggtcgcatggcggcttcaggggtttgggtctcgtggcgtaccagaaggtggtgagtgctgcaaaagctccgaagcccataagcgtgttggtcggaagagtacgcacgtactgtcggaagtcaaccagctctggcattcgaaaataccggaacagctcatgggcttgcattgtcctgtgttgatagttctctaagctgaattcgactgggggaacgcctgtccccagactcgaatccacgtgtccattcaagtcatctaccgccactctccgtctcctccgtggaccggccgctccgccgccggctgtcactgcagcccactccct

SEQ ID NO: 9083 - RNA, 2248 nt, Homo sapiens
  source 1..2248: mol_type = other RNA
actggacttggagtcagaaggccattgtcgatagaaaataattcagggtgcaatgtgatgcctttgacctgttcaaatggtttcagaccagaatccttcccaagtctcaccatatcttcgaggatagcttttttgacatccttatttctgcacagttcctcaaacgacccttcaaatcctctcttttgggcccaggaacataatgtctcaacatctggtaccacaattgcaatgagaaatgcctgcaggctttctccgtggacaaacacctgagcaacaggctcacttcgcatgtagatattttcaatcttttcaggggctatgtattctccttgtgccagcttaaatatgtgctttttccggtcgataattttcaaggtgccatttggtaaccattttccaatgtcccctgtgtgtaaccagccgtctttgtccaaagcttctgctgttttcgctgggtccttcaagtagccctgaaatacatttggccctttcacacacacctcgccctcgccctcggcagccatgtaattcatttcttccacatcaacaagttttatcaaattgcacggcatcggggccccaacatggcctgcggtccagtctccaggcatggtcaggcagcacccggcagtgcactctgtctgtccgtatccttcataaaactgacagcccagggctgctctgaggaacgtcagcacagtggcagacaccggggcggctcctgtcaccatcagccggactcttccgcccaggctcgactgtactttgtggaagatcagccggtcccacaggctgttgtttctgatgatgccgctgcgaagctctgcttctttcctcttggaggcaaagtccaagagccatcgcttcagcgtggtgtttgcttgtccgaaaattcggtcaaacatccggttcagcagtcttggaaccacggggaagacagtgggttgaagcaccttgaggtcatccatgagcagcctgatatctccttggaaaaatccgattttagctccatgacacagcattacacactctacaactctctcaaacatatgggcgagaggcaagaaagatatcaaagtatcatctgggcaaggattgactgtattctctgttgctttcacaaaagctgaacaatcgctcactatgtttcggtgagtgaccattgctcctttggggttgcctgtagttccacttgtgaaacaaattactgcaagatcttcaggtgctggaggcttgggcttccgtctgttggctcttcccaggtcctccatcgccttcatgctggtgacttccaccccacacctctggcctcgttccaccagttcactgccgtaggcatccatgacaactatgattttaaggcctggtattaacttattttctacaccctctaataagagtttggccttctctggcttgtcaacaaaaaccagagagagttcagctttgttgactatgtacgtgatggcttcatttccaagggtatcataaagtggaacgatcaccatcgaataagcaaagcatccttgttcaataatcacccactcaggtctattttgagcaaagatgccaatgaactgatctggggcagtcttgaagcccttctggatcagtgctgagcctatgcactccgacaattctgcaacctgtttatatgaaagccattcatagggttggtctggtttccgagagcctaaacaagggccattatttgacacctgtattcccctctggaaaccttcgtataatgttgtgacatcatcatagaaatacaccaagggctcgtcgctgtcaagtagtgcggatcttcgtgcaccaccactacccgccacttccactgactgcatggagaggtcgcatggcggcttcaggggtttgggtctcgtggcgtaccagaaggtggtgagtgctgcaaaagctccgaagcccataagcgtgttggtcggaagagtacgcacgtactgtcggaagtcaaccagctctggcattcgaaaataccggaacagctcatgggcttgcattgtcctgtgttgatagttctctaagctgaattctagatcctggggtcctctcaggtgctctgcccaaagtcaggatcttcccatcttcccgtggtgaaaggttttctttgccttcagcaagtttaggatatcaatgaagacaaacacacctgcaagagttaacagagctacagaagacagatctgataaccacggcaggtagggccctggtgctccaggaatct

SEQ ID NO: 9084 - RNA, 2174 nt, Homo sapiens
  source 1..2174: mol_type = other RNA
actggacttggagtcagaaggccattgtcgatagaaaataattcagggtgcaatgtgatgcctttgacctgttcaaatggtttcagaccagaatccttcccaagtctcaccatatcttcgaggatagcttttttgacatccttatttctgcacagttcctcaaacgacccttcaaatcctctcttttgggcccaggaacataatgtctcaacatctggtaccacaattgcaatgagaaatgcctgcaggctttctccgtggacaaacacctgagcaacaggctcacttcgcatgtagatattttcaatcttttcaggggctatgtattctccttgtgccagcttaaatatgtgctttttccggtcgataattttcaaggtgccatttggtaaccattttccaatgtcccctgtgtgtaaccagccgtctttgtccaaagcttctgctgttttcgctgggtccttcaagtagccctgaaatacatttggccctttcacacacacctcgccctcgccctcggcagccatgtaattcatttcttccacatcaacaagttttatcaaattgcacggcatcggggccccaacatggcctgcggtccagtctccaggcatggtcaggcagcacccggcagtgcactctgtctgtccgtatccttcataaaactgacagcccagggctgctctgaggaacgtcagcacagtggcagacaccggggcggctcctgtcaccatcagccggactcttccgcccaggctcgactgtactttgtggaagatcagccggtcccacaggctgttgtttctgatgatgccgctgcgaagctctgcttctttcctcttggaggcaaagtccaagagccatcgcttcagcgtggtgtttgcttgtccgaaaattcggtcaaacatccggttcagcagtcttggaaccacggggaagacagtgggttgaagcaccttgaggtcatccatgagcagcctgatatctccttggaaaaatccgattttagctccatgacacagcattacacactctacaactctctcaaacatatgggcgagaggcaagaaagatatcaaagtatcatctgggcaaggattgactgtattctctgttgctttcacaaaagctgaacaatcgctcactatgtttcggtgagtgaccattgctcctttggggttgcctgtagttccacttgtgaaacaaattactgcaagatcttcaggtgctggaggcttgggcttccgtctgttggctcttcccaggtcctccatcgccttcatgctggtgacttccaccccacacctctggcctcgttccaccagttcactgccgtaggcatccatgacaactatgattttaaggcctggtattaacttattttctacaccctctaataagagtttggccttctctggcttgtcaacaaaaaccagagagagttcagctttgttgactatgtacgtgatggcttcatttccaagggtatcataaagtggaacgatcaccatcgaataagcaaagcatccttgttcaataatcacccactcaggtctattttgagcaaagatgccaatgaactgatctggggcagtcttgaagcccttctggatcagtgctgagcctatgcactccgacaattctgcaacctgtttatatgaaagccattcatagggttggtctggtttccgagagcctaaacaagggccattatttgacacctgtattcccctctggaaaccttcgtataatgttgtgacatcatcatagaaatacaccaagggctcgtcgctgtcaagtagtgcggatcttcgtgcaccaccactacccgccacttccactgactgcatggagaggtcgcatggcggcttcaggggtttgggtctcgtggcgtaccagaaggtggtgagtgctgcaaaagctccgaagcccataagcgtgttggtcggaagagtacgcacgtactgtcggaagtcaaccagctctggcattcgaaaataccggaacagctcatgggcttgcattgtcctgtgttgatagttctctaagctgaattctagatcctggggtcctctcaggtgctctgcccaaagtcaggatcttcccatcttcccgtggtgactcctccgtggaccggccgctccgccgccggctgtcactgcagcccactccct

SEQ ID NO: 9085 - RNA, 2109 nt, Homo sapiens
  source 1..2109: mol_type = other RNA
actggacttggagtcagaaggccattgtcgatagaaaataattcagggtgcaatgtgatgcctttgacctgttcaaatggtttcagaccagaatccttcccaagtctcaccatatcttcgaggatagcttttttgacatccttatttctgcacagttcctcaaacgacccttcaaatcctctcttttgggcccaggaacataatgtctcaacatctggtaccacaattgcaatgagaaatgcctgcaggctttctccgtggacaaacacctgagcaacaggctcacttcgcatgtagatattttcaatcttttcaggggctatgtattctccttgtgccagcttaaatatgtgctttttccggtcgataattttcaaggtgccatttggtaaccattttccaatgtcccctgtgtgtaaccagccgtctttgtccaaagcttctgctgttttcgctgggtccttcaagtagccctgaaatacatttggccctttcacacacacctcgccctcgccctcggcagccatgtaattcatttcttccacatcaacaagttttatcaaattgcacggcatcggggccccaacatggcctgcggtccagtctccaggcatggtcaggcagcacccggcagtgcactctgtctgtccgtatccttcataaaactgacagcccagggctgctctgaggaacgtcagcacagtggcagacaccggggcggctcctgtcaccatcagccggactcttccgcccaggctcgactgtactttgtggaagatcagccggtcccacaggctgttgtttctgatgatgccgctgcgaagctctgcttctttcctcttggaggcaaagtccaagagccatcgcttcagcgtggtgtttgcttgtccgaaaattcggtcaaacatccggttcagcagtcttggaaccacggggaagacagtgggttgaagcaccttgaggtcatccatgagcagcctgatatctccttggaaaaatccgattttagctccatgacacagcattacacactctacaactctctcaaacatatgggcgagaggcaagaaagatatcaaagtatcatctgggcaaggattgactgtattctctgttgctttcacaaaagctgaacaatcgctcactatgtttcggtgagtgaccattgctcctttggggttgcctgtagttccacttgtgaaacaaattactgcaagatcttcaggtgctggaggcttgggcttccgtctgttggctcttcccaggtcctccatcgccttcatgctggtgacttccaccccacacctctggcctcgttccaccagttcactgccgtaggcatccatgacaactatgattttaaggcctggtattaacttattttctacaccctctaataagagtttggccttctctggcttgtcaacaaaaaccagagagagttcagctttgttgactatgtacgtgatggcttcatttccaagggtatcataaagtggaacgatcaccatcgaataagcaaagcatccttgttcaataatcacccactcaggtctattttgagcaaagatgccaatgaactgatctggggcagtcttgaagcccttctggatcagtgctgagcctatgcactccgacaattctgcaacctgtttatatgaaagccattcatagggttggtctggtttccgagagcctaaacaagggccattatttgacacctgtattcccctctggaaaccttcgtataatgttgtgacatcatcatagaaatacaccaagggctcgtcgctgtcaagtagtgcggatcttcgtgcaccaccactacccgccacttccactgactgcatggagaggtcgcatggcggcttcaggggtttgggtctcgtggcgtaccagaaggtggtgagtgctgcaaaagctccgaagcccataagcgtgttggtcggaagagtacgcacgtactgtcggaagtcaaccagctctggcattcgaaaataccggaacagctcatgggcttgcattgtcctgtgttgatagttctctaagctgaattctcctccgtggaccggccgctccgccgccggctgtcactgcagcccactccct

SEQ ID NO: 9086 - RNA, 2125 nt, Homo sapiens
  source 1..2125: mol_type = other RNA
actggacttggagtcagaaggccattgtcgatagaaaataattcagggtgcaatgtgatgcctttgacctgttcaaatggtttcagaccagaatccttcccaagtctcaccatatcttcgaggatagcttttttgacatccttatttctgcacagttcctcaaacgacccttcaaatcctctcttttgggcccaggaacataatgtctcaacatctggtaccacaattgcaatgagaaatgcctgcaggctttctccgtggacaaacacctgagcaacaggctcacttcgcatgtagatattttcaatcttttcaggggctatgtattctccttgtgccagcttaaatatgtgctttttccggtcgataattttcaaggtgccatttggtaaccattttccaatgtcccctgtgtgtaaccagccgtctttgtccaaagcttctgctgttttcgctgggtccttcaagtagccctgaaatacatttggccctttcacacacacctcgccctcgccctcggcagccatgtaattcatttcttccacatcaacaagttttatcaaattgcacggcatcggggccccaacatggcctgcggtccagtctccaggcatggtcaggcagcacccggcagtgcactctgtctgtccgtatccttcataaaactgacagcccagggctgctctgaggaacgtcagcacagtggcagacaccggggcggctcctgtcaccatcagccggactcttccgcccaggctcgactgtactttgtggaagatcagccggtcccacaggctgttgtttctgatgatgccgctgcgaagctctgcttctttcctcttggaggcaaagtccaagagccatcgcttcagcgtggtgtttgcttgtccgaaaattcggtcaaacatccggttcagcagtcttggaaccacggggaagacagtgggttgaagcaccttgaggtcatccatgagcagcctgatatctccttggaaaaatccgattttagctccatgacacagcattacacactctacaactctctcaaacatatgggcgagaggcaagaaagatatcaaagtatcatctgggcaaggattgactgtattctctgttgctttcacaaaagctgaacaatcgctcactatgtttcggtgagtgaccattgctcctttggggttgcctgtagttccacttgtgaaacaaattactgcaagatcttcaggtgctggaggcttgggcttccgtctgttggctcttcccaggtcctccatcgccttcatgctggtgacttccaccccacacctctggcctcgttccaccagttcactgccgtaggcatccatgacaactatgattttaaggcctggtattaacttattttctacaccctctaataagagtttggccttctctggcttgtcaacaaaaaccagagagagttcagctttgttgactatgtacgtgatggcttcatttccaagggtatcataaagtggaacgatcaccatcgaataagcaaagcatccttgttcaataatcacccactcaggtctattttgagcaaagatgccaatgaactgatctggggcagtcttgaagcccttctggatcagtgctgagcctatgcactccgacaattctgcaacctgtttatatgaaagccattcatagggttggtctggtttccgagagcctaaacaagggccattatttgacacctgtattcccctctggaaaccttcgtataatgttgtgacatcatcatagaaatacaccaagggctcgtcgctgtcaagtagtgcggatcttcgtgcaccaccactacccgccacttccactgactgcatggagaggtcgcatggcggcttcaggggtttgggtctcgtggcgtaccagaaggtggtgagtgctgcaaaagctccgaagcccataagcgtgttggtcggaagagtacgcacgtactgtcggaagtcaaccagctctggcattcgaaaataccggaacagctcatgggcttgcattgtcctgtgttgatagttctctaagctgaattcttttctgtctggtgtctgcagagcctgacgtgggcagcgcccgcagctcgcgccggtgcaggggagct

SEQ ID NO: 9087 - RNA, 1882 nt, Homo sapiens
  source 1..1882: mol_type = other RNA
actggacttggagtcagaaggccattgtcgatagaaaataattcagggtgcaatgtgatgcctttgacctgttcaaatggtttcagaccagaatccttcccaagtctcaccatatcttcgaggatagcttttttgacatccttatttctgcacagttcctcaaacgacccttcaaatcctctcttttgggcccaggaacataatgtctcaacatctggtaccacaattgcaatgagaaatgcctgcaggctttctccgtggacaaacacctgagcaacaggctcacttcgcatgtagatattttcaatcttttcaggggctatgtattctccttgtgccagcttaaatatgtgctttttccggtcgataattttcaaggtgccatttggtaaccattttccaatgtcccctgtgtgtaaccagccgtctttgtccaaagcttctgctgttttcgctgggtccttcaagtagccctgaaatacatttggccctttcacacacacctcgccctcgccctcggcagccatgtaattcatttcttccacatcaacaagttttatcaaattgcacggcatcggggccccaacatggcctgcggtccagtctccaggcatggtcaggcagcacccggcagtgcactctgtctgtccgtatccttcataaaactgacagcccagggctgctctgaggaacgtcagcacagtggcagacaccggggcggctcctgtcaccatcagccggactcttccgcccaggctcgactgtactttgtggaagatcagccggtcccacaggctgttgtttctgatgatgccgctgcgaagctctgcttctttcctcttggaggcaaagtccaagagccatcgcttcagcgtggtgtttgcttgtccgaaaattcggtcaaacatccggttcagcagtcttggaaccacggggaagacagtgggttgaagcaccttgaggtcatccatgagcagcctgatatctccttggaaaaatccgattttagctccatgacacagcattacacactctacaactctctcaaacatatgggcgagaggcaagaaagatatcaaagtatcatctgggcaaggattgactgtattctctgttgctttcacaaaagctgaacaatcgctcactatgtttcggtgagtgaccattgctcctttggggttgcctgtagttccacttgtgaaacaaattactgcaagatcttcaggtgctggaggcttgggcttccgtctgttggctcttcccaggtcctccatcgccttcatgctggtgacttccaccccacacctctggcctcgttccaccagttcactgccgtaggcatccatgacaactatgattttaaggcctggtattaacttattttctacaccctctaataagagtttggccttctctggcttgtcaacaaaaaccagagagagttcagctttgttgactatgtacgtgatggcttcatttccaagggtatcataaagtggaacgatcaccatcgaataagcaaagcatccttgttcaataatcacccactcaggtctattttgagcaaagatgccaatgaactgatctggggcagtcttgaagcccttctggatcagtgctgagcctatgcactccgacaattctgcaacctgtttatatgaaagccattcatagggttggtctggtttccgagagcctaaacaagggccattatttgacacctgtattcccctctggaaaccttcgtataatgttgtgacatcatcatagaaatacaccaagggctcgtcgctgtcaagtagtgcggatcttcgtgcaccaccactaccctcctccgtggaccggccgctccgccgccggctgtcactgcagcccactccct

SEQ ID NO: 9088 - RNA, 2007 nt, Homo sapiens
  source 1..2007: mol_type = other RNA
actggacttggagtcagaaggccattgtcgatagaaaataattcagggtgcaatgtgatgcctttgacctgttcaaatggtttcagaccagaatccttcccaagtctcaccatatcttcgaggatagcttttttgacatccttatttctgcacagttcctcaaacgacccttcaaatcctctcttttgggcccaggaacataatgtctcaacatctggtaccacaattgcaatgagaaatgcctgcaggctttctccgtggacaaacacctgagcaacaggctcacttcgcatgtagatattttcaatcttttcaggggctatgtattctccttgtgccagcttaaatatgtgctttttccggtcgataattttcaaggtgccatttggtaaccattttccaatgtcccctgtgtgtaaccagccgtctttgtccaaagcttctgctgttttcgctgggtccttcaagtagccctgaaatacatttggccctttcacacacacctcgccctcgccctcggcagccatgtaattcatttcttccacatcaacaagttttatcaaattgcacggcatcggggccccaacatggcctgcggtccagtctccaggcatggtcaggcagcacccggcagtgcactctgtctgtccgtatccttcataaaactgacagcccagggctgctctgaggaacgtcagcacagtggcagacaccggggcggctcctgtcaccatcagccggactcttccgcccaggctcgactgtactttgtggaagatcagccggtcccacaggctgttgtttctgatgatgccgctgcgaagctctgcttctttcctcttggaggcaaagtccaagagccatcgcttcagcgtggtgtttgcttgtccgaaaattcggtcaaacatccggttcagcagtcttggaaccacggggaagacagtgggttgaagcaccttgaggtcatccatgagcagcctgatatctccttggaaaaatccgattttagctccatgacacagcattacacactctacaactctctcaaacatatgggcgagaggcaagaaagatatcaaagtatcatctgggcaaggattgactgtattctctgttgctttcacaaaagctgaacaatcgctcactatgtttcggtgagtgaccattgctcctttggggttgcctgtagttccacttgtgaaacaaattactgcaagatcttcaggtgctggaggcttgggcttccgtctgttggctcttcccaggtcctccatcgccttcatgctggtgacttccaccccacacctctggcctcgttccaccagttcactgccgtaggcatccatgacaactatgattttaaggcctggtattaacttattttctacaccctctaataagagtttggccttctctggcttgtcaacaaaaaccagagagagttcagctttgttgactatgtacgtgatggcttcatttccaagggtatcataaagtggaacgatcaccatcgaataagcaaagcatccttgttcaataatcacccactgtttatatgaaagccattcatagggttggtctggtttccgagagcctaaacaagggccattatttgacacctgtattcccctctggaaaccttcgtataatgttgtgacatcatcatagaaatacaccaagggctcgtcgctgtcaagtagtgcggatcttcgtgcaccaccactacccgccacttccactgactgcatggagaggtcgcatggcggcttcaggggtttgggtctcgtggcgtaccagaaggtggtgagtgctgcaaaagctccgaagcccataagcgtgttggtcggaagagtacgcacgtactgtcggaagtcaaccagctctggcattcgaaaataccggaacagctcatgggcttgcattgtcctgtgttgatagttctctaagctgaattctcctccgtggaccggccgctccgccgccggctgtcactgcagcccactccct

SEQ ID NO: 9089 - RNA, 2306 nt, Homo sapiens
  source 1..2306: mol_type = other RNA
actggacttggagtcagaaggccattgtcgatagaaaataattcagggtgcaatgtgatgcctttgacctgttcaaatggtttcagaccagaatccttcccaagtctcaccatatcttcgaggatagcttttttgacatccttatttctgcacagttcctcaaacgacccttcaaatcctctcttttgggcccaggaacataatgtctcaacatctggtaccacaattgcaatgagaaatgcctgcaggctttctccgtggacaaacacctgagcaacaggctcacttcgcatgtagatattttcaatcttttcaggggctatgtattctccttgtgccagcttaaatatgtgctttttccggtcgataattttcaaggtgccatttggtaaccattttccaatgtcccctgtgtgtaaccagccgtctttgtccaaagcttctgctgttttcgctgggtccttcaagtagccctgaaatacatttggccctttcacacacacctcgccctcgccctcggcagccatgtaattcatttcttccacatcaacaagttttatcaaattgcacggcatcggggccccaacatggcctgcggtccagtctccaggcatggtcaggcagcacccggcagtgcactctgtctgtccgtatccttcataaaactgacagcccagggctgctctgaggaacgtcagcacagtggcagacaccggggcggctcctgtcaccatcagccggactcttccgcccaggctcgactgtactttgtggaagatcagccggtcccacaggctgttgtttctgatgatgccgctgcgaagctctgcttctttcctcttggaggcaaagtccaagagccatcgcttcagcgtggtgtttgcttgtccgaaaattcggtcaaacatccggttcagcagtcttggaaccacggggaagacagtgggttgaagcaccttgaggtcatccatgagcagcctgatatctccttggaaaaatccgattttagctccatgacacagcattacacactctacaactctctcaaacatatgggcgagaggcaagaaagatatcaaagtatcatctgggcaaggattgactgtattctctgttgctttcacaaaagctgaacaatcgctcactatgtttcggtgagtgaccattgctcctttggggttgcctgtagttccacttgtgaaacaaattactgcaagatcttcaggtgctggaggcttgggcttccgtctgttggctcttcccaggtcctccatcgccttcatgctggtgacttccaccccacacctctggcctcgttccaccagttcactgccgtaggcatccatgacaactatgattttaaggcctggtattaacttattttctacaccctctaataagagtttggccttctctggcttgtcaacaaaaaccagagagagttcagctttgttgactatgtacgtgatggcttcatttccaagggtatcataaagtggaacgatcaccatcgaataagcaaagcatccttgttcaataatcacccatggttcatacctcaggtctattttgagcaaagatgccaatgaactgatctggggcagtcttgaagcccttctggatcagtgctgagcctatgcactccgacaattctgcaacctgtttatatgaaagccattcatagggttggtctggtttccgagagcctaaacaagggccattatttgacacctgtattcccctctggaaaccttcgtataatgttgtgacatcatcatagaaatacaccaagggctcgtcgctgtcaagtagtgcggatcttcgtgcaccaccactacccgccacttccactgactgcatggagaggtcgcatggcggcttcaggggtttgggtctcgtggcgtaccagaaggtggtgagtgctgcaaaagctccgaagcccataagcgtgttggtcggaagagtacgcacgtactgtcggaagtcaaccagctctggcattcgaaaataccggaacagctcatgggcttgcattgtcctgtgttgatagttctctaagctgaattattaacattgtattctcttcatgtcatttagaaaccaaaaaccgggtggtctggatgtttctctccttctaaagttcctcaagctttcatcaagatgaataatggcagtttgatggaatacttcactaggaatgcagccctcaaacaaacccacataaatgacacccttgcccctgcagtggcaaattaagaaagcctgacatctttccttaacgcagcaacccaagctggcaagatgct

SEQ ID NO: 9090 - RNA, 2093 nt, Homo sapiens
  source 1..2093: mol_type = other RNA
actggacttggagtcagaaggccattgtcgatagaaaataattcagggtgcaatgtgatgcctttgacctgttcaaatggtttcagaccagaatccttcccaagtctcaccatatcttcgaggatagcttttttgacatccttatttctgcacagttcctcaaacgacccttcaaatcctctcttttgggcccaggaacataatgtctcaacatctggtaccacaattgcaatgagaaatgcctgcaggctttctccgtggacaaacacctgagcaacaggctcacttcgcatgtagatattttcaatcttttcaggggctatgtattctccttgtgccagcttaaatatgtgctttttccggtcgataattttcaaggtgccatttggtaaccattttccaatgtcccctgtgtgtaaccagccgtctttgtccaaagcttctgctgttttcgctgggtccttcaagtagccctgaaatacatttggccctttcacacacacctcgccctcgccctcggcagccatgtaattcatttcttccacatcaacaagttttatcaaattgcacggcatcggggccccaacatggcctgcggtccagtctccaggcatggtcaggcagcacccggcagtgcactctgtctgtccgtatccttcataaaactgacagcccagggctgctctgaggaacgtcagcacagtggcagacaccggggcggctcctgtcaccatcagccggactcttccgcccaggctcgactgtactttgtggaagatcagccggtcccacaggctgttgtttctgatgatgccgctgcgaagctctgcttctttcctcttggaggcaaagtccaagagccatcgcttcagcgtggtgtttgcttgtccgaaaattcggtcaaacatccggttcagcagtcttggaaccacggggaagacagtgggttgaagcaccttgaggtcatccatgagcagcctgatatctccttggaaaaatccgattttagctccatgacacagcattacacactctacaactctctcaaacatatgggcgagaggcaagaaagatatcaaagtatcatctgggcaaggattgactgtattctctgttgctttcacaaaagctgaacaatcgctcactatgtttcggtgagtgaccattgctcctttggggttgcctgtagttccacttgtgaaacaaattactgcaagatcttcaggtgctggaggcttgggcttccgtctgttggctcttcccaggtcctccatcgccttcatgctggtgacttccaccccacacctctggcctcgttccaccagttcactgccgtaggcatccatgacaactatgattttaaggcctggtattaacttattttctacaccctctaataagagtttggccttctctggcttgtcaacaaaaaccagagagagttcagctttgttgactatgtacgtgatggcttcatttccaagggtatcataaagtggaacgatcaccatcgaataagcaaagcatccttgttcaataatcacccatggttcatacctcaggtctattttgagcaaagatgccaatgaactgatctggggcagtcttgaagcccttctggatcagtgctgagcctatgcactccgacaattctgcaacctgtttatatgaaagccattcatagggttggtctggtttccgagagcctaaacaagggccattatttgacacctgtattcccctctggaaaccttcgtataatgttgtgacatcatcatagaaatacaccaagggctcgtcgctgtcaagtagtgcggatcttcgtgcaccaccactacccgccacttccactgactgcatggagaggtcgcatggcggcttcaggggtttgggtctcgtggcgtaccagaaggtggtgagtgctgcaaaagctccgaagcccataagcgtgttggtcggaagagtacgcacgtactgtcggaagtcaaccagctctggcattcgaaaataccggaacagctcatgggcttgcattgtcctgtgttgatagttctctaagctgaattcatctgtgccaccaacagctgactact

SEQ ID NO: 9091 - RNA, 2119 nt, Homo sapiens
  source 1..2119: mol_type = other RNA
actggacttggagtcagaaggccattgtcgatagaaaataattcagggtgcaatgtgatgcctttgacctgttcaaatggtttcagaccagaatccttcccaagtctcaccatatcttcgaggatagcttttttgacatccttatttctgcacagttcctcaaacgacccttcaaatcctctcttttgggcccaggaacataatgtctcaacatctggtaccacaattgcaatgagaaatgcctgcaggctttctccgtggacaaacacctgagcaacaggctcacttcgcatgtagatattttcaatcttttcaggggctatgtattctccttgtgccagcttaaatatgtgctttttccggtcgataattttcaaggtgccatttggtaaccattttccaatgtcccctgtgtgtaaccagccgtctttgtccaaagcttctgctgttttcgctgggtccttcaagtagccctgaaatacatttggccctttcacacacacctcgccctcgccctcggcagccatgtaattcatttcttccacatcaacaagttttatcaaattgcacggcatcggggccccaacatggcctgcggtccagtctccaggcatggtcaggcagcacccggcagtgcactctgtctgtccgtatccttcataaaactgacagcccagggctgctctgaggaacgtcagcacagtggcagacaccggggcggctcctgtcaccatcagccggactcttccgcccaggctcgactgtactttgtggaagatcagccggtcccacaggctgttgtttctgatgatgccgctgcgaagctctgcttctttcctcttggaggcaaagtccaagagccatcgcttcagcgtggtgtttgcttgtccgaaaattcggtcaaacatccggttcagcagtcttggaaccacggggaagacagtgggttgaagcaccttgaggtcatccatgagcagcctgatatctccttggaaaaatccgattttagctccatgacacagcattacacactctacaactctctcaaacatatgggcgagaggcaagaaagatatcaaagtatcatctgggcaaggattgactgtattctctgttgctttcacaaaagctgaacaatcgctcactatgtttcggtgagtgaccattgctcctttggggttgcctgtagttccacttgtgaaacaaattactgcaagatcttcaggtgctggaggcttgggcttccgtctgttggctcttcccaggtcctccatcgccttcatgctggtgacttccaccccacacctctggcctcgttccaccagttcactgccgtaggcatccatgacaactatgattttaaggcctggtattaacttattttctacaccctctaataagagtttggccttctctggcttgtcaacaaaaaccagagagagttcagctttgttgactatgtacgtgatggcttcatttccaagggtatcataaagtggaacgatcaccatcgaataagcaaagcatccttgttcaataatcacccatggttcatacctcaggtctattttgagcaaagatgccaatgaactgatctggggcagtcttgaagcccttctggatcagtgctgagcctatgcactccgacaattctgcaacctgtttatatgaaagccattcatagggttggtctggtttccgagagcctaaacaagggccattatttgacacctgtattcccctctggaaaccttcgtataatgttgtgacatcatcatagaaatacaccaagggctcgtcgctgtcaagtagtgcggatcttcgtgcaccaccactacccgccacttccactgactgcatggagaggtcgcatggcggcttcaggggtttgggtctcgtggcgtaccagaaggtggtgagtgctgcaaaagctccgaagcccataagcgtgttggtcggaagagtacgcacgtactgtcggaagtcaaccagctctggcattcgaaaataccggaacagctcatgggcttgcattgtcctgtgttgatagttctctaagctgaattctcctccgtggaccggccgctccgccgccggctgtcactgcagcccactccct

SEQ ID NO: 9092 - RNA, 1892 nt, Homo sapiens
  source 1..1892: mol_type = other RNA
actggacttggagtcagaaggccattgtcgatagaaaataattcagggtgcaatgtgatgcctttgacctgttcaaatggtttcagaccagaatccttcccaagtctcaccatatcttcgaggatagcttttttgacatccttatttctgcacagttcctcaaacgacccttcaaatcctctcttttgggcccaggaacataatgtctcaacatctggtaccacaattgcaatgagaaatgcctgcaggctttctccgtggacaaacacctgagcaacaggctcacttcgcatgtagatattttcaatcttttcaggggctatgtattctccttgtgccagcttaaatatgtgctttttccggtcgataattttcaaggtgccatttggtaaccattttccaatgtcccctgtgtgtaaccagccgtctttgtccaaagcttctgctgttttcgctgggtccttcaagtagccctgaaatacatttggccctttcacacacacctcgccctcgccctcggcagccatgtaattcatttcttccacatcaacaagttttatcaaattgcacggcatcggggccccaacatggcctgcggtccagtctccaggcatggtcaggcagcacccggcagtgcactctgtctgtccgtatccttcataaaactgacagcccagggctgctctgaggaacgtcagcacagtggcagacaccggggcggctcctgtcaccatcagccggactcttccgcccaggctcgactgtactttgtggaagatcagccggtcccacaggctgttgtttctgatgatgccgctgcgaagctctgcttctttcctcttggaggcaaagtccaagagccatcgcttcagcgtggtgtttgcttgtccgaaaattcggtcaaacatccggttcagcagtcttggaaccacggggaagacagtgggttgaagcaccttgaggtcatccatgagcagcctgatatctccttggaaaaatccgattttagctccatgacacagcattacacactctacaactctctcaaacatatgggcgagaggcaagaaagatatcaaagtatcatctgggcaaggattgactgtattctctgttgctttcacaaaagctgaacaatcgctcactatgtttcggtgagtgaccattgctcctttggggttgcctgtagttccacttgtgaaacaaattactgcaagatcttcaggtgctggaggcttgggcttccgtctgttggctcttcccaggtcctccatcgccttcatgctggtgacttccaccccacacctctggcctcgttccaccagttcactgccgtaggcatccatgacaactatgattttaaggcctggtattaacttattttctacaccctctaataagagtttggccttctctggcttgtcaacaaaaaccagagagagttcagctttgttgactatgtacgtgatggcttcatttccaagggtatcataaagtggaacgatcaccatcgaataagcaaagcatccttgttcaataatcacccatggttcatacctcaggtctattttgagcaaagatgccaatgaactgatctggggcagtcttgaagcccttctggatcagtgctgagcctatgcactccgacaattctgcaacctgtttatatgaaagccattcatagggttggtctggtttccgagagcctaaacaagggccattatttgacacctgtattcccctctggaaaccttcgtataatgttgtgacatcatcatagaaatacaccaagggctcgtcgctgtcaagtagtgcggatcttcgtgcaccaccactaccctcctccgtggaccggccgctccgccgccggctgtcactgcagcccactccct

SEQ ID NO: 9093 - RNA, 2155 nt, Homo sapiens
  source 1..2155: mol_type = other RNA
actggacttggagtcagaaggccattgtcgatagaaaataattcagggtgcaatgtgatgcctttgacctgttcaaatggtttcagaccagaatccttcccaagtctcaccatatcttcgaggatagcttttttgacatccttatttctgcacagttcctcaaacgacccttcaaatcctctcttttgggcccaggaacataatgtctcaacatctggtaccacaattgcaatgagaaatgcctgcaggctttctccgtggacaaacacctgagcaacaggctcacttcgcatgtagatattttcaatcttttcaggggctatgtattctccttgtgccagcttaaatatgtgctttttccggtcgataattttcaaggtgccatttggtaaccattttccaatgtcccctgtgtgtaaccagccgtctttgtccaaagcttctgctgttttcgctgggtccttcaagtagccctgaaatacatttggccctttcacacacacctcgccctcgccctcggcagccatgtaattcatttcttccacatcaacaagttttatcaaattgcacggcatcggggccccaacatggcctgcggtccagtctccaggcatggtcaggcagcacccggcagtgcactctgtctgtccgtatccttcataaaactgacagcccagggctgctctgaggaacgtcagcacagtggcagacaccggggcggctcctgtcaccatcagccggactcttccgcccaggctcgactgtactttgtggaagatcagccggtcccacaggctgttgtttctgatgatgccgctgcgaagctctgcttctttcctcttggaggcaaagtccaagagccatcgcttcagcgtggtgtttgcttgtccgaaaattcggtcaaacatccggttcagcagtcttggaaccacggggaagacagtgggttgaagcaccttgaggtcatccatgagcagcctgatatctccttggaaaaatccgattttagctccatgacacagcattacacactctacaactctctcaaacatatgggcgagaggcaagaaagatatcaaagtatcatctgggcaaggattgactgtattctctgttgctttcacaaaagctgaacaatcgctcactatgtttcggtgagtgaccattgctcctttggggttgcctgtagttccacttgtgaaacaaattactgcaagatcttcaggtgctggaggcttgggcttccgtctgttggctcttcccaggtcttctttatcatacagcagtcaaaaaacaccagaaaaattcttgcatctccatcgccttcatgctggtgacttccaccccacacctctggcctcgttccaccagttcactgccgtaggcatccatgacaactatgattttaaggcctggtattaacttattttctacaccctctaataagagtttggccttctctggcttgtcaacaaaaaccagagagagttcagctttgttgactatgtacgtgatggcttcatttccaagggtatcataaagtggaacgatcaccatcgaataagcaaagcatccttgttcaataatcacccactcaggtctattttgagcaaagatgccaatgaactgatctggggcagtcttgaagcccttctggatcagtgctgagcctatgcactccgacaattctgcaacctgtttatatgaaagccattcatagggttggtctggtttccgagagcctaaacaagggccattatttgacacctgtattcccctctggaaaccttcgtataatgttgtgacatcatcatagaaatacaccaagggctcgtcgctgtcaagtagtgcggatcttcgtgcaccaccactacccgccacttccactgactgcatggagaggtcgcatggcggcttcaggggtttgggtctcgtggcgtaccagaaggtggtgagtgctgcaaaagctccgaagcccataagcgtgttggtcggaagagtacgcacgtactgtcggaagtcaaccagctctggcattcgaaaataccggaacagctcatgggcttgcattgtcctgtgttgatagttctctaagctgaattctcctccgtggaccggccgctccgccgccggctgtcactgcagcccactccct

SEQ ID NO: 9094 - RNA, 2296 nt, Homo sapiens
  source 1..2296: mol_type = other RNA
actggacttggagtcagaaggccattgtcgatagaaaataattcagggtgcaatgtgatgcctttgacctgttcaaatggtttcagaccagaatccttcccaagtctcaccatatcttcgaggatagcttttttgacatccttatttctgcacagttcctcaaacgacccttcaaatcctctcttttgggcccaggaacataatgtctcaacatctggtaccacaattgcaatgagaaatgcctgcaggctttctccgtggacaaacacctgagcaacaggctcacttcgcatgtagatattttcaatcttttcaggggctatgtattctccttgtgccagcttaaatatgtgctttttccggtcgataattttcaaggtgccatttggtaaccattttccaatgtcccctgtgtgtaaccagccgtctttgtccaaagcttctgctgttttcgctgggtccttcaagtagccctgaaatacatttggccctttcacacacacctcgccctcgccctcggcagccatgtaattcatttcttccacatcaacaagttttatcaaattgcacggcatcggggccccaacatggcctgcggtccagtctccaggcatggtcaggcagcacccggcagtgcactctgtctgtccgtatccttcataaaactgacagcccagggctgctctgaggaacgtcagcacagtggcagacaccggggcggctcctgtcaccatcagccggactcttccgcccaggctcgactgtactttgtggaagatcagccggtcccacaggctgttgtttctgatgatgccgctgcgaagctctgcttctttcctcttggaggcaaagtccaagagccatcgcttcagcgtggtgtttgcttgtccgaaaattcggtcaaacatccggttcagcagtcttggaaccacggggaagacagtgggttgaagcaccttgaggtcatccatgagcagcctgatatctccttggaaaaatccgattttagctccatgacacagcattacacacttcaataactgttcataaatgtgagcaagtggtaaatatgaaatgtgtgtgtcactggcactcaagggaagtgctttctctgttgctttcacaaaagctgaacaatcgctcactatgtttcggtgagtgaccattgctcctttggggttgcctgtagttccacttgtgaaacaaattactgcaagatcttcaggtgctggaggcttgggcttccgtctgttggctcttcccaggtcctccatcgccttcatgctggtgacttccaccccacacctctggcctcgttccaccagttcactgccgtaggcatccatgacaactatgattttaaggcctggtattaacttattttctacaccctctaataagagtttggccttctctggcttgtcaacaaaaaccagagagagttcagctttgttgactatgtacgtgatggcttcatttccaagggtatcataaagtggaacgatcaccatcgaataagcaaagcatccttgttcaataatcacccactcaggtctattttgagcaaagatgccaatgaactgatctggggcagtcttgaagcccttctggatcagtgctgagcctatgcactccgacaattctgcaacctgtttatatgaaagccattcatagggttggtctggtttccgagagcctaaacaagggccattatttgacacctgtattcccctctggaaaccttcgtataatgttgtgacatcatcatagaaatacaccaagggctcgtcgctgtcaagtagtgcggatcttcgtgcaccaccactacccgccacttccactgactgcatggagaggtcgcatggcggcttcaggggtttgggtctcgtggcgtaccagaaggtggtgagtgctgcaaaagctccgaagcccataagcgtgttggtcggaagagtacgcacgtactgtcggaagtcaaccagctctggcattcgaaaataccggaacagctcatgggcttgcattgtcctgtgttgatagttctctaagctgaattattaacattgtattctcttcatgtcatttagaaaccaaaaaccgggtggtctggatgtttctctccttctaaagttcctcaagctttcatcaagatgaataatggcagtttgatggaatacttcactaggaatgcagccctcaaacaaacccacataaatgacacccttgcccctgcagtggcaaattaagaaagcctgacatctttccttaacgcagcaacccaagctggcaagatgct

SEQ ID NO: 9095 - RNA, 2083 nt, Homo sapiens
  source 1..2083: mol_type = other RNA
actggacttggagtcagaaggccattgtcgatagaaaataattcagggtgcaatgtgatgcctttgacctgttcaaatggtttcagaccagaatccttcccaagtctcaccatatcttcgaggatagcttttttgacatccttatttctgcacagttcctcaaacgacccttcaaatcctctcttttgggcccaggaacataatgtctcaacatctggtaccacaattgcaatgagaaatgcctgcaggctttctccgtggacaaacacctgagcaacaggctcacttcgcatgtagatattttcaatcttttcaggggctatgtattctccttgtgccagcttaaatatgtgctttttccggtcgataattttcaaggtgccatttggtaaccattttccaatgtcccctgtgtgtaaccagccgtctttgtccaaagcttctgctgttttcgctgggtccttcaagtagccctgaaatacatttggccctttcacacacacctcgccctcgccctcggcagccatgtaattcatttcttccacatcaacaagttttatcaaattgcacggcatcggggccccaacatggcctgcggtccagtctccaggcatggtcaggcagcacccggcagtgcactctgtctgtccgtatccttcataaaactgacagcccagggctgctctgaggaacgtcagcacagtggcagacaccggggcggctcctgtcaccatcagccggactcttccgcccaggctcgactgtactttgtggaagatcagccggtcccacaggctgttgtttctgatgatgccgctgcgaagctctgcttctttcctcttggaggcaaagtccaagagccatcgcttcagcgtggtgtttgcttgtccgaaaattcggtcaaacatccggttcagcagtcttggaaccacggggaagacagtgggttgaagcaccttgaggtcatccatgagcagcctgatatctccttggaaaaatccgattttagctccatgacacagcattacacacttcaataactgttcataaatgtgagcaagtggtaaatatgaaatgtgtgtgtcactggcactcaagggaagtgctttctctgttgctttcacaaaagctgaacaatcgctcactatgtttcggtgagtgaccattgctcctttggggttgcctgtagttccacttgtgaaacaaattactgcaagatcttcaggtgctggaggcttgggcttccgtctgttggctcttcccaggtcctccatcgccttcatgctggtgacttccaccccacacctctggcctcgttccaccagttcactgccgtaggcatccatgacaactatgattttaaggcctggtattaacttattttctacaccctctaataagagtttggccttctctggcttgtcaacaaaaaccagagagagttcagctttgttgactatgtacgtgatggcttcatttccaagggtatcataaagtggaacgatcaccatcgaataagcaaagcatccttgttcaataatcacccactcaggtctattttgagcaaagatgccaatgaactgatctggggcagtcttgaagcccttctggatcagtgctgagcctatgcactccgacaattctgcaacctgtttatatgaaagccattcatagggttggtctggtttccgagagcctaaacaagggccattatttgacacctgtattcccctctggaaaccttcgtataatgttgtgacatcatcatagaaatacaccaagggctcgtcgctgtcaagtagtgcggatcttcgtgcaccaccactacccgccacttccactgactgcatggagaggtcgcatggcggcttcaggggtttgggtctcgtggcgtaccagaaggtggtgagtgctgcaaaagctccgaagcccataagcgtgttggtcggaagagtacgcacgtactgtcggaagtcaaccagctctggcattcgaaaataccggaacagctcatgggcttgcattgtcctgtgttgatagttctctaagctgaattcatctgtgccaccaacagctgactact

SEQ ID NO: 9096 - RNA, 2170 nt, Homo sapiens
  source 1..2170: mol_type = other RNA
actggacttggagtcagaaggccattgtcgatagaaaataattcagggtgcaatgtgatgcctttgacctgttcaaatggtttcagaccagaatccttcccaagtctcaccatatcttcgaggatagcttttttgacatccttatttctgcacagttcctcaaacgacccttcaaatcctctcttttgggcccaggaacataatgtctcaacatctggtaccacaattgcaatgagaaatgcctgcaggctttctccgtggacaaacacctgagcaacaggctcacttcgcatgtagatattttcaatcttttcaggggctatgtattctccttgtgccagcttaaatatgtgctttttccggtcgataattttcaaggtgccatttggtaaccattttccaatgtcccctgtgtgtaaccagccgtctttgtccaaagcttctgctgttttcgctgggtccttcaagtagccctgaaatacatttggccctttcacacacacctcgccctcgccctcggcagccatgtaattcatttcttccacatcaacaagttttatcaaattgcacggcatcggggccccaacatggcctgcggtccagtctccaggcatggtcaggcagcacccggcagtgcactctgtctgtccgtatccttcataaaactgacagcccagggctgctctgaggaacgtcagcacagtggcagacaccggggcggctcctgtcaccatcagccggactcttccgcccaggctcgactgtactttgtggaagatcagccggtcccacaggctgttgtttctgatgatgccgctgcgaagctctgcttctttcctcttggaggcaaagtccaagagccatcgcttcagcgtggtgtttgcttgtccgaaaattcggtcaaacatccggttcagcagtcttggaaccacggggaagacagtgggttgaagcaccttgaggtcatccatgagcagcctgatatctccttggaaaaatccgattttagctccatgacacagcattacacacttcaataactgttcataaatgtgagcaagtggtaaatatgaaatgtgtgtgtcactggcactcaagggaagtgctttctctgttgctttcacaaaagctgaacaatcgctcactatgtttcggtgagtgaccattgctcctttggggttgcctgtagttccacttgtgaaacaaattactgcaagatcttcaggtgctggaggcttgggcttccgtctgttggctcttcccaggtcctccatcgccttcatgctggtgacttccaccccacacctctggcctcgttccaccagttcactgccgtaggcatccatgacaactatgattttaaggcctggtattaacttattttctacaccctctaataagagtttggccttctctggcttgtcaacaaaaaccagagagagttcagctttgttgactatgtacgtgatggcttcatttccaagggtatcataaagtggaacgatcaccatcgaataagcaaagcatccttgttcaataatcacccactcaggtctattttgagcaaagatgccaatgaactgatctggggcagtcttgaagcccttctggatcagtgctgagcctatgcactccgacaattctgcaacctgtttatatgaaagccattcatagggttggtctggtttccgagagcctaaacaagggccattatttgacacctgtattcccctctggaaaccttcgtataatgttgtgacatcatcatagaaatacaccaagggctcgtcgctgtcaagtagtgcggatcttcgtgcaccaccactacccgccacttccactgactgcatggagaggtcgcatggcggcttcaggggtttgggtctcgtggcgtaccagaaggtggtgagtgctgcaaaagctccgaagcccataagcgtgttggtcggaagagtacgcacgtactgtcggaagtcaaccagctctggcattcgaaaataccggaacagctcatgggcttgcattgtcctgtgttgatagttctctaagctgaattcatgacagcaaagaaagaacagataagcagatttcttcaggccatggttctggaaagaaggcaccagcacttaacaaaaccactcaccatctgtgccaccaacagctgactact

SEQ ID NO: 9097 - RNA, 2174 nt, Homo sapiens
  source 1..2174: mol_type = other RNA
actggacttggagtcagaaggccattgtcgatagaaaataattcagggtgcaatgtgatgcctttgacctgttcaaatggtttcagaccagaatccttcccaagtctcaccatatcttcgaggatagcttttttgacatccttatttctgcacagttcctcaaacgacccttcaaatcctctcttttgggcccaggaacataatgtctcaacatctggtaccacaattgcaatgagaaatgcctgcaggctttctccgtggacaaacacctgagcaacaggctcacttcgcatgtagatattttcaatcttttcaggggctatgtattctccttgtgccagcttaaatatgtgctttttccggtcgataattttcaaggtgccatttggtaaccattttccaatgtcccctgtgtgtaaccagccgtctttgtccaaagcttctgctgttttcgctgggtccttcaagtagccctgaaatacatttggccctttcacacacacctcgccctcgccctcggcagccatgtaattcatttcttccacatcaacaagttttatcaaattgcacggcatcggggccccaacatggcctgcggtccagtctccaggcatggtcaggcagcacccggcagtgcactctgtctgtccgtatccttcataaaactgacagcccagggctgctctgaggaacgtcagcacagtggcagacaccggggcggctcctgtcaccatcagccggactcttccgcccaggctcgactgtactttgtggaagatcagccggtcccacaggctgttgtttctgatgatgccgctgcgaagctctgcttctttcctcttggaggcaaagtccaagagccatcgcttcagcgtggtgtttgcttgtccgaaaattcggtcaaacatccggttcagcagtcttggaaccacggggaagacagtgggttgaagcaccttgaggtcatccatgagcagcctgatatctccttggaaaaatccgattttagctccatgacacagcattacacacttcaataactgttcataaatgtgagcaagtggtaaatatgaaatgtgtgtgtcactggcactcaagggaagtgctttctctgttgctttcacaaaagctgaacaatcgctcactatgtttcggtgagtgaccattgctcctttggggttgcctgtagttccacttgtgaaacaaattactgcaagatcttcaggtgctggaggcttgggcttccgtctgttggctcttcccaggtcctccatcgccttcatgctggtgacttccaccccacacctctggcctcgttccaccagttcactgccgtaggcatccatgacaactatgattttaaggcctggtattaacttattttctacaccctctaataagagtttggccttctctggcttgtcaacaaaaaccagagagagttcagctttgttgactatgtacgtgatggcttcatttccaagggtatcataaagtggaacgatcaccatcgaataagcaaagcatccttgttcaataatcacccactcaggtctattttgagcaaagatgccaatgaactgatctggggcagtcttgaagcccttctggatcagtgctgagcctatgcactccgacaattctgcaacctgtttatatgaaagccattcatagggttggtctggtttccgagagcctaaacaagggccattatttgacacctgtattcccctctggaaaccttcgtataatgttgtgacatcatcatagaaatacaccaagggctcgtcgctgtcaagtagtgcggatcttcgtgcaccaccactacccgccacttccactgactgcatggagaggtcgcatggcggcttcaggggtttgggtctcgtggcgtaccagaaggtggtgagtgctgcaaaagctccgaagcccataagcgtgttggtcggaagagtacgcacgtactgtcggaagtcaaccagctctggcattcgaaaataccggaacagctcatgggcttgcattgtcctgtgttgatagttctctaagctgaattctagatcctggggtcctctcaggtgctctgcccaaagtcaggatcttcccatcttcccgtggtgactcctccgtggaccggccgctccgccgccggctgtcactgcagcccactccct

SEQ ID NO: 9098 - RNA, 2109 nt, Homo sapiens
  source 1..2109: mol_type = other RNA
actggacttggagtcagaaggccattgtcgatagaaaataattcagggtgcaatgtgatgcctttgacctgttcaaatggtttcagaccagaatccttcccaagtctcaccatatcttcgaggatagcttttttgacatccttatttctgcacagttcctcaaacgacccttcaaatcctctcttttgggcccaggaacataatgtctcaacatctggtaccacaattgcaatgagaaatgcctgcaggctttctccgtggacaaacacctgagcaacaggctcacttcgcatgtagatattttcaatcttttcaggggctatgtattctccttgtgccagcttaaatatgtgctttttccggtcgataattttcaaggtgccatttggtaaccattttccaatgtcccctgtgtgtaaccagccgtctttgtccaaagcttctgctgttttcgctgggtccttcaagtagccctgaaatacatttggccctttcacacacacctcgccctcgccctcggcagccatgtaattcatttcttccacatcaacaagttttatcaaattgcacggcatcggggccccaacatggcctgcggtccagtctccaggcatggtcaggcagcacccggcagtgcactctgtctgtccgtatccttcataaaactgacagcccagggctgctctgaggaacgtcagcacagtggcagacaccggggcggctcctgtcaccatcagccggactcttccgcccaggctcgactgtactttgtggaagatcagccggtcccacaggctgttgtttctgatgatgccgctgcgaagctctgcttctttcctcttggaggcaaagtccaagagccatcgcttcagcgtggtgtttgcttgtccgaaaattcggtcaaacatccggttcagcagtcttggaaccacggggaagacagtgggttgaagcaccttgaggtcatccatgagcagcctgatatctccttggaaaaatccgattttagctccatgacacagcattacacacttcaataactgttcataaatgtgagcaagtggtaaatatgaaatgtgtgtgtcactggcactcaagggaagtgctttctctgttgctttcacaaaagctgaacaatcgctcactatgtttcggtgagtgaccattgctcctttggggttgcctgtagttccacttgtgaaacaaattactgcaagatcttcaggtgctggaggcttgggcttccgtctgttggctcttcccaggtcctccatcgccttcatgctggtgacttccaccccacacctctggcctcgttccaccagttcactgccgtaggcatccatgacaactatgattttaaggcctggtattaacttattttctacaccctctaataagagtttggccttctctggcttgtcaacaaaaaccagagagagttcagctttgttgactatgtacgtgatggcttcatttccaagggtatcataaagtggaacgatcaccatcgaataagcaaagcatccttgttcaataatcacccactcaggtctattttgagcaaagatgccaatgaactgatctggggcagtcttgaagcccttctggatcagtgctgagcctatgcactccgacaattctgcaacctgtttatatgaaagccattcatagggttggtctggtttccgagagcctaaacaagggccattatttgacacctgtattcccctctggaaaccttcgtataatgttgtgacatcatcatagaaatacaccaagggctcgtcgctgtcaagtagtgcggatcttcgtgcaccaccactacccgccacttccactgactgcatggagaggtcgcatggcggcttcaggggtttgggtctcgtggcgtaccagaaggtggtgagtgctgcaaaagctccgaagcccataagcgtgttggtcggaagagtacgcacgtactgtcggaagtcaaccagctctggcattcgaaaataccggaacagctcatgggcttgcattgtcctgtgttgatagttctctaagctgaattctcctccgtggaccggccgctccgccgccggctgtcactgcagcccactccct

SEQ ID NO: 9099 - RNA, 1882 nt, Homo sapiens
  source 1..1882: mol_type = other RNA
actggacttggagtcagaaggccattgtcgatagaaaataattcagggtgcaatgtgatgcctttgacctgttcaaatggtttcagaccagaatccttcccaagtctcaccatatcttcgaggatagcttttttgacatccttatttctgcacagttcctcaaacgacccttcaaatcctctcttttgggcccaggaacataatgtctcaacatctggtaccacaattgcaatgagaaatgcctgcaggctttctccgtggacaaacacctgagcaacaggctcacttcgcatgtagatattttcaatcttttcaggggctatgtattctccttgtgccagcttaaatatgtgctttttccggtcgataattttcaaggtgccatttggtaaccattttccaatgtcccctgtgtgtaaccagccgtctttgtccaaagcttctgctgttttcgctgggtccttcaagtagccctgaaatacatttggccctttcacacacacctcgccctcgccctcggcagccatgtaattcatttcttccacatcaacaagttttatcaaattgcacggcatcggggccccaacatggcctgcggtccagtctccaggcatggtcaggcagcacccggcagtgcactctgtctgtccgtatccttcataaaactgacagcccagggctgctctgaggaacgtcagcacagtggcagacaccggggcggctcctgtcaccatcagccggactcttccgcccaggctcgactgtactttgtggaagatcagccggtcccacaggctgttgtttctgatgatgccgctgcgaagctctgcttctttcctcttggaggcaaagtccaagagccatcgcttcagcgtggtgtttgcttgtccgaaaattcggtcaaacatccggttcagcagtcttggaaccacggggaagacagtgggttgaagcaccttgaggtcatccatgagcagcctgatatctccttggaaaaatccgattttagctccatgacacagcattacacacttcaataactgttcataaatgtgagcaagtggtaaatatgaaatgtgtgtgtcactggcactcaagggaagtgctttctctgttgctttcacaaaagctgaacaatcgctcactatgtttcggtgagtgaccattgctcctttggggttgcctgtagttccacttgtgaaacaaattactgcaagatcttcaggtgctggaggcttgggcttccgtctgttggctcttcccaggtcctccatcgccttcatgctggtgacttccaccccacacctctggcctcgttccaccagttcactgccgtaggcatccatgacaactatgattttaaggcctggtattaacttattttctacaccctctaataagagtttggccttctctggcttgtcaacaaaaaccagagagagttcagctttgttgactatgtacgtgatggcttcatttccaagggtatcataaagtggaacgatcaccatcgaataagcaaagcatccttgttcaataatcacccactcaggtctattttgagcaaagatgccaatgaactgatctggggcagtcttgaagcccttctggatcagtgctgagcctatgcactccgacaattctgcaacctgtttatatgaaagccattcatagggttggtctggtttccgagagcctaaacaagggccattatttgacacctgtattcccctctggaaaccttcgtataatgttgtgacatcatcatagaaatacaccaagggctcgtcgctgtcaagtagtgcggatcttcgtgcaccaccactaccctcctccgtggaccggccgctccgccgccggctgtcactgcagcccactccct

SEQ ID NO: 9100 - RNA, 5654 nt, Homo sapiens
  source 1..5654: mol_type = other RNA
actggacttggagtcagaaggcctaataatcagtccctaaaatcaagtggcaactactgatattgcaggatagtgcctaggaaagaattaagagacccaaagggttgaccttgcagagactccagcctatgaagtatcagcaagtgccaaaaatttatggctctgcaaaaaagcacagggtgactcaattatgcagagagctctaccacccaatgcaaaaccctggctcccggaatctaaaggacgaaatgttgcttaaagtatgatatattaacaattccagtgcttaaaagtttccctcactaaatatttctcttggatgtaccttagcaagctcttaggaagttgctgagtgttctgatgctggtcctgtgtcctttccactttctatcgtctacttcccagctcctgtgctttccttccagagagaactgtgtgtgcagtgtactttctatgcttcaccttcagggaccttctcttctttcctttctctgtctttgtccttgagctgtgttgtctgcactgctgaatggtggcagtcctgctgcaaggttgttgttcatagattgtatgacaccagcctcaacgggtgactgtgggaactagagttagaaatctgaagctcttctgcaaagtgccttgaactcttgatagggaagatgctattgaaagggacaaattcttttaaaagtaaatattgtggcagaagtctttgttgataaaatgacacaatgcagtaacagcttcagatctggggtaaaatcagatgccaatttccatctgaacacacgatgatcctgtgttgcatcattacacatttttacttcgtgtaaaaatttctaagcaaactaatactcaaaattaatgcaagtataatgaaagtttatcattcagatttattgccatataataaatctttcacaaaaatcaggaagaagcctctggtgactttgcagagctgaggcagtgatgcacgtggtggggcctccctcctgagcgggaaccaggactgggagcatcacttgcaggcctccatggaggctgctgccccagctgagctgttagctagtgagtgcttctactgtgtgatgaatgagaaaagggaaagaggggagggcaatcagggttctgggggcacctcagtgagcccagaggcctggaggagaggctgtatgattccccagtcaggccttccttgggagtgtgccctctgtcaagatgactgggtttttgaagggcctcatttcctcacacaacaagcactgacagtcctgcagcccagggactgtcctgtggcactgcccagccctcagactcagaggacagttctgtggtcctgccagaagctcagctgttccacatgacccttaaacatttaaacaattttttggtttaaaggaaaaggaagccaatcaaaatgctttggaaacaaattaaagttgcaaattatttccccacatagtaaatacatatccttgctacctgaaatgataatcatcactccccctgctggctgagagcgcttctcctccttcagactggctctgccacaaagctaagtattagtagaagttgttgccaagcctcacctctagcctgtacatgggctctgaggtgaacacaggagtcagagtccccactccagcagtgactggaggaggcctgacagaacaagccccttggggacaggaggcaagctgcactcacctctgggaccccacccgggatgggcgctccacgagtcccttggccttagggaacctctgtttcattccatccagacgaggatagggaagcttcctgccctacctcgacagcctctaagagcacagcttggccaggccttcccgtgtggagcccacacagtggtgcactgagaggctgccagtgttttgaccttttacagagcttggggtgactgagaatggttcctccgaggccctcggaagatttgatggactcaaataacacgggcctgcagccctgggacacaggacaggagaagccagccctgacacagatgagctggcagtggattcgaacagtgtgctcagtctcgtctgggcttttgtgctttctatgttgaagaccaaatactttttctttgagaatgaaactaggctccttatctagactgtgaaggggcccgtgaggacacagagtgtgactggaaaggaaggtcccaactggccctcaatgtggccccagtggctgtttccctgcaagaagctccttcctccagctcaggcaccaacacacggatcacaccggcccagaaacaaagagcaaaacatgcttttcatcccacgtggaatacagtatgaacaaattactctcctttttctattagtgtgggtgaaggaaaaagactgttttcaaatgaagcttttctttttcccaatgattaatacagagtagattaacttaatttgtgctagactccaatttaattccagcaacagttcacaggccatattcacagaaaagttaatctgggcttcatgagaagtagccattttctttttcttttctttctttttttttttttgcgagacagggtctcactttgtggctcaggctggagtgtactggcacgttcttagctcactgcagccttgaactcctgggctcaggcaatcctcctaccttagcctcctgagtagctaggactacaggaatgtgccatcatgcctggctaatttttaagttttttgtagagatgggatctcactatgttgcccaagctggtttcagattcctgtgctcaagggattctgctaacttggctccccaaagtgctgggattacaaatgtgagccactgtatctggcccatattcttttttaagaaaagatgcagaggtgttaaatattaatatcaaattgtccaggcatggtgtttatgaaattgtgtgccctctgacaggcaaccaaacacacacgacttcatttctttattaattcctgcctcatcatcttttctcattgatgctccttaatgtcaaaggaatctctctctctcacacacacataagaccaaaacaaatatcttgaacatgcaaaaaaatagtctacgcttttgaatagtgtgcactgttgaatagtgtgcactgttggatagtgtgcactgttgaagtgtgatgtgcctaaggcaacaggatcttgggaaagctctagatttttggcttcgaaataaaactgcatgttgaatagcaggtttttacatttattattgttgtgtatttcctcccctttttgcaatactatctacgctgagttatctattgccaactagcaccaattctccaaatcaaagtgtgtgaggaaaacacactcgtgcaatcctctttaacagaagatacaccaagtaacctgtctgtctacttctgttacccagaaataaaagaacttgaagggctgcttggctggaggggtccgggtgggagagcatcctgccctcagtcggaatccatggtgaacagctggatgtcctgtggattccagtacaggccgactgctgagttgtagacaagagaccagacataggggataaaaaactcctcgggctgctcctcttccacatatttgaatttcaattctggaaatttcagatcaatattttgcattatatcctgaaatgaaggatgagttcgaaattgttcaaagagatcgcgtttgtaaagcagggcgtataccaagtttgggttgtggtgaagggaatttgtcaggcaggagttgatgatctctaacatcattcgaatcacttcttcaatgacatttaggtcttgtgcataatctggtagaggaacatcattagaactcagcgaacctctcaaggactgtgtggcttgttccagaactttgttgtgttttttagacagcaaagaaaataaactgatgatcctctgggcagcatactgatggagagaacgaaactgtgccgacatatttgctaaagctgccaaacaatttgtgtgaaggtacttgtctcgtgtcctagtcatgttgtattgaatggttcttattaccaccaggatcaggagactccccaaggagatttcagttaaaactcgttctgaataccaagtaatattttttagtatcacttcatgaatggatctgttgaagccatcatcttccgtaaggatcaacaatattataagggccatatacacatggtgtgaattcctttcttcaacatgatacagaatctcaagaattggtaaaacaagattttccatatctgtgcgagccaacatgtatgttctaatattactattttgatggagcaaggtatacaagaggagagttgcttgatcagatgtctgctgttcacaaagagctgtgtacaaactattaaagttgatctggaaggcatgtggaattgatgaggggaaaggactgctatcttgtgtgttcttgaaggacataatggcttgtctgtaggggtttggcgcatctgaggcatctgtcagattggccaacaccagcagaagcaggagactctggttggccagaggggaagaaagctctggagaggcagccgctttgctgcccacaccacctagtgtgaagacagtccagagtcctgttgctactcctgatgcaagtccataaagcagtcctcccccatccgactgctgagggaaaacatgggcccctggaggaggtggcttttcttgtctgataaagttatataataaggtcttcacaagtttgctggtgtatggaagacatggacctcgcatcaaatacttgtggctgatgctctgtcgcaaaacttctttgtggaagagttggcaggaaaggaaaacaaccattgttgatatagcttctactgatatttcatatgtaatatctaagagtggaatatcagtgatcaactgcatcaaacagcacagcaattcttccaaaagatcttctgagtcagaactgtaattgccaggagatttttcttcataagtaaaatgaagttgtaattcctcctctgacatctgacagatgaacactttcagcaaacagcaaataataaacaaagcattgtgtgtctgccaaatgaagatgtggttctgacattctgctgaaagttttagttctttggttctagaaaggaagaccttaattagtgcaccaagatttcctgttcgaggattgttttcaactaatgacctgcagactgaaatggttgcttcctccaagagtttcaactcactactgctagttggtgcagggaaagaaaatgagagaagctgattccagaacgggtcattctcagagatagattccgtgcctgataactttttcaagtactcatttttaggaagatcgccgattctgctgctattcgatcccatcttctagcttaagcagataatttgtccttaaacctgcatttccaaaagacaacctgtctcagccggctgggggatctgctccagctccacggacccgcggacggatgggagggtggcagaggggtcaggagaagtcgctgtcgccgccgcagcccaggtggcgcacaccggctcaggcctccatgtttccacgtctcagcgggtacagatccggctccggtccggcctgcagctcggccccggctcggctccagcccgggccgcgtcggtgcggaggccaggaggcggcgagagaagaggg

SEQ ID NO: 9101 - RNA, 5651 nt, Homo sapiens
  source 1..5651: mol_type = other RNA
actggacttggagtcagaaggcctaataatcagtccctaaaatcaagtggcaactactgatattgcaggatagtgcctaggaaagaattaagagacccaaagggttgaccttgcagagactccagcctatgaagtatcagcaagtgccaaaaatttatggctctgcaaaaaagcacagggtgactcaattatgcagagagctctaccacccaatgcaaaaccctggctcccggaatctaaaggacgaaatgttgcttaaagtatgatatattaacaattccagtgcttaaaagtttccctcactaaatatttctcttggatgtaccttagcaagctcttaggaagttgctgagtgttctgatgctggtcctgtgtcctttccactttctatcgtctacttcccagctcctgtgctttccttccagagagaactgtgtgtgcagtgtactttctatgcttcaccttcagggaccttctcttctttcctttctctgtctttgtccttgagctgtgttgtctgcactgctgaatggtggcagtcctgctgcaaggttgttgttcatagattgtatgacaccagcctcaacgggtgactgtgggaactagagttagaaatctgaagctcttctgcaaagtgccttgaactcttgatagggaagatgctattgaaagggacaaattcttttaaaagtaaatattgtggcagaagtctttgttgataaaatgacacaatgcagtaacagcttcagatctggggtaaaatcagatgccaatttccatctgaacacacgatgatcctgtgttgcatcattacacatttttacttcgtgtaaaaatttctaagcaaactaatactcaaaattaatgcaagtataatgaaagtttatcattcagatttattgccatataataaatctttcacaaaaatcaggaagaagcctctggtgactttgcagagctgaggcagtgatgcacgtggtggggcctccctcctgagcgggaaccaggactgggagcatcacttgcaggcctccatggaggctgctgccccagctgagctgttagctagtgagtgcttctactgtgtgatgaatgagaaaagggaaagaggggagggcaatcagggttctgggggcacctcagtgagcccagaggcctggaggagaggctgtatgattccccagtcaggccttccttgggagtgtgccctctgtcaagatgactgggtttttgaagggcctcatttcctcacacaacaagcactgacagtcctgcagcccagggactgtcctgtggcactgcccagccctcagactcagaggacagttctgtggtcctgccagaagctcagctgttccacatgacccttaaacatttaaacaattttttggtttaaaggaaaaggaagccaatcaaaatgctttggaaacaaattaaagttgcaaattatttccccacatagtaaatacatatccttgctacctgaaatgataatcatcactccccctgctggctgagagcgcttctcctccttcagactggctctgccacaaagctaagtattagtagaagttgttgccaagcctcacctctagcctgtacatgggctctgaggtgaacacaggagtcagagtccccactccagcagtgactggaggaggcctgacagaacaagccccttggggacaggaggcaagctgcactcacctctgggaccccacccgggatgggcgctccacgagtcccttggccttagggaacctctgtttcattccatccagacgaggatagggaagcttcctgccctacctcgacagcctctaagagcacagcttggccaggccttcccgtgtggagcccacacagtggtgcactgagaggctgccagtgttttgaccttttacagagcttggggtgactgagaatggttcctccgaggccctcggaagatttgatggactcaaataacacgggcctgcagccctgggacacaggacaggagaagccagccctgacacagatgagctggcagtggattcgaacagtgtgctcagtctcgtctgggcttttgtgctttctatgttgaagaccaaatactttttctttgagaatgaaactaggctccttatctagactgtgaaggggcccgtgaggacacagagtgtgactggaaaggaaggtcccaactggccctcaatgtggccccagtggctgtttccctgcaagaagctccttcctccagctcaggcaccaacacacggatcacaccggcccagaaacaaagagcaaaacatgcttttcatcccacgtggaatacagtatgaacaaattactctcctttttctattagtgtgggtgaaggaaaaagactgttttcaaatgaagcttttctttttcccaatgattaatacagagtagattaacttaatttgtgctagactccaatttaattccagcaacagttcacaggccatattcacagaaaagttaatctgggcttcatgagaagtagccattttctttttcttttctttctttttttttttttgcgagacagggtctcactttgtggctcaggctggagtgtactggcacgttcttagctcactgcagccttgaactcctgggctcaggcaatcctcctaccttagcctcctgagtagctaggactacaggaatgtgccatcatgcctggctaatttttaagttttttgtagagatgggatctcactatgttgcccaagctggtttcagattcctgtgctcaagggattctgctaacttggctccccaaagtgctgggattacaaatgtgagccactgtatctggcccatattcttttttaagaaaagatgcagaggtgttaaatattaatatcaaattgtccaggcatggtgtttatgaaattgtgtgccctctgacaggcaaccaaacacacacgacttcatttctttattaattcctgcctcatcatcttttctcattgatgctccttaatgtcaaaggaatctctctctctcacacacacataagaccaaaacaaatatcttgaacatgcaaaaaaatagtctacgcttttgaatagtgtgcactgttgaatagtgtgcactgttggatagtgtgcactgttgaagtgtgatgtgcctaaggcaacaggatcttgggaaagctctagatttttggcttcgaaataaaactgcatgttgaatagcaggtttttacatttattattgttgtgtatttcctcccctttttgcaatactatctacgctgagttatctattgccaactagcaccaattctccaaatcaaagtgtgtgaggaaaacacactcgtgcaatcctctttaacagaagatacaccaagtaacctgtctgtctacttctgttacccagaaataaaagaacttgaagggctgcttggctggaggggtccgggtgggagagcatcctgccctcagtcggaatccatggtgaacagctggatgtcctgtggattccagtacaggccgactgctgagttgtagacaagagaccagacataggggataaaaaactcctcgggctgctcctcttccacatatttgaatttcaattctggaaatttcagatcaatattttgcattatatcctgaaatgaaggatgagttcgaaattgttcaaagagatcgcgtttgtaaagcagggcgtataccaagtttgggttgtggtgaagggaatttgtcaggcaggagttgatgatctctaacatcattcgaatcacttcttcaatgacatttaggtcttgtgcataatctggtagaggaacatcattagaactcagcgaacctctcaaggactgtgtggcttgttccagaactttgttgtgttttttagacagcaaagaaaataaactgatgatcctctgggcagcatactgatggagagaacgaaactgtgccgacatatttgctaaagctgccaaacaatttgtgtgaaggtacttgtctcgtgtcctagtcatgttgtattgaatggttcttattaccaccaggatcaggagactccccaaggagatttcagttaaaactcgttctgaataccaagtaatattttttagtatcacttcatgaatggatctgttgaagccatcatcttccgtaaggatcaacaatattataagggccatatacacatggtgtgaattcctttcttcaacatgatacagaatctcaagaattggtaaaacaagattttccatatctgtgcgagccaacatgtatgttctaatattactattttgatggagcaaggtatacaagaggagagttgcttgatcagatgtctgctgttcacaaagagctgtgtacaaactattaaagttgatctggaaggcatgtggaattgatgaggggaaaggactgctatcttgtgtgttcttgaaggacataatggcttgtctgtaggggtttggcgcatctgaggcatctgtcagattggccaacaccagcagaagcaggagactctggttggccagaggggaagaaagctctggagaggcagccgctttgctgcccacaccacctagtgtgaagacagtccagagtcttgctactcctgatgcaagtccataaagcagtcctcccccatccgactgctgagggaaaacatgggcccctggaggaggtggcttttcttgtctgataaagttatataataaggtcttcacaagtttgctggtgtatggaagacatggacctcgcatcaaatacttgtggctgatgctctgtcgcaaaacttctttgtggaagagttggcaggaaaggaaaacaaccattgttgatatagcttctactgatatttcatatgtaatatctaagagtggaatatcagtgatcaactgcatcaaacagcacagcaattcttccaaaagatcttctgagtcagaactgtaattgccaggagatttttcttcataagtaaaatgaagttgtaattcctcctctgacatctgacagatgaacactttcagcaaacagcaaataataaacaaagcattgtgtgtctgccaaatgaagatgtggttctgacattctgctgaaagttttagttctttggttctagaaaggaagaccttaattagtgcaccaagatttcctgttcgaggattgttttcaactaatgacctgcagactgaaatggttgcttcctccaagagtttcaactcactactgctagttggtgcagggaaagaaaatgagagaagctgattccagaacgggtcattctcagagatagattccgtgcctgataactttttcaagtactcatttttaggaagatcgccgattctgctgctattcgatcccatcttctagcttaagcagataatttgtccttaaacctgcatttccaaaagacaacctgtctcagccggctgggggatctgctccagctccacggacccgcggacggatgggagggtggcagaggggtcaggagaagtcgctgtcgccgccgcagcccaggtggcgcacaccggctcaggcctccatgtttccacgtctcagcgggtacagatccggctccggtccggcctgcagctcggccccggctcggctccagcccgggccgcgtcggtgcggaggccaggaggcggcgagagaagaggg

SEQ ID NO: 9102 - RNA, 5819 nt, Homo sapiens
  source 1..5819: mol_type = other RNA
actggacttggagtcagaaggcctaataatcagtccctaaaatcaagtggcaactactgatattgcaggatagtgcctaggaaagaattaagagacccaaagggttgaccttgcagagactccagcctatgaagtatcagcaagtgccaaaaatttatggctctgcaaaaaagcacagggtgactcaattatgcagagagctctaccacccaatgcaaaaccctggctcccggaatctaaaggacgaaatgttgcttaaagtatgatatattaacaattccagtgcttaaaagtttccctcactaaatatttctcttggatgtaccttagcaagctcttaggaagttgctgagtgttctgatgctggtcctgtgtcctttccactttctatcgtctacttcccagctcctgtgctttccttccagagagaactgtgtgtgcagtgtactttctatgcttcaccttcagggaccttctcttctttcctttctctgtctttgtccttgagctgtgttgtctgcactgctgaatggtggcagtcctgctgcaaggttgttgttcatagattgtatgacaccagcctcaacgggtgactgtgggaactagagttagaaatctgaagctcttctgcaaagtgccttgaactcttgatagggaagatgctattgaaagggacaaattcttttaaaagtaaatattgtggcagaagtctttgttgataaaatgacacaatgcagtaacagcttcagatctggggtaaaatcagatgccaatttccatctgaacacacgatgatcctgtgttgcatcattacacatttttacttcgtgtaaaaatttctaagcaaactaatactcaaaattaatgcaagtataatgaaagtttatcattcagatttattgccatataataaatctttcacaaaaatcaggaagaagcctctggtgactttgcagagctgaggcagtgatgcacgtggtggggcctccctcctgagcgggaaccaggactgggagcatcacttgcaggcctccatggaggctgctgccccagctgagctgttagctagtgagtgcttctactgtgtgatgaatgagaaaagggaaagaggggagggcaatcagggttctgggggcacctcagtgagcccagaggcctggaggagaggctgtatgattccccagtcaggccttccttgggagtgtgccctctgtcaagatgactgggtttttgaagggcctcatttcctcacacaacaagcactgacagtcctgcagcccagggactgtcctgtggcactgcccagccctcagactcagaggacagttctgtggtcctgccagaagctcagctgttccacatgacccttaaacatttaaacaattttttggtttaaaggaaaaggaagccaatcaaaatgctttggaaacaaattaaagttgcaaattatttccccacatagtaaatacatatccttgctacctgaaatgataatcatcactccccctgctggctgagagcgcttctcctccttcagactggctctgccacaaagctaagtattagtagaagttgttgccaagcctcacctctagcctgtacatgggctctgaggtgaacacaggagtcagagtccccactccagcagtgactggaggaggcctgacagaacaagccccttggggacaggaggcaagctgcactcacctctgggaccccacccgggatgggcgctccacgagtcccttggccttagggaacctctgtttcattccatccagacgaggatagggaagcttcctgccctacctcgacagcctctaagagcacagcttggccaggccttcccgtgtggagcccacacagtggtgcactgagaggctgccagtgttttgaccttttacagagcttggggtgactgagaatggttcctccgaggccctcggaagatttgatggactcaaataacacgggcctgcagccctgggacacaggacaggagaagccagccctgacacagatgagctggcagtggattcgaacagtgtgctcagtctcgtctgggcttttgtgctttctatgttgaagaccaaatactttttctttgagaatgaaactaggctccttatctagactgtgaaggggcccgtgaggacacagagtgtgactggaaaggaaggtcccaactggccctcaatgtggccccagtggctgtttccctgcaagaagctccttcctccagctcaggcaccaacacacggatcacaccggcccagaaacaaagagcaaaacatgcttttcatcccacgtggaatacagtatgaacaaattactctcctttttctattagtgtgggtgaaggaaaaagactgttttcaaatgaagcttttctttttcccaatgattaatacagagtagattaacttaatttgtgctagactccaatttaattccagcaacagttcacaggccatattcacagaaaagttaatctgggcttcatgagaagtagccattttctttttcttttctttctttttttttttttgcgagacagggtctcactttgtggctcaggctggagtgtactggcacgttcttagctcactgcagccttgaactcctgggctcaggcaatcctcctaccttagcctcctgagtagctaggactacaggaatgtgccatcatgcctggctaatttttaagttttttgtagagatgggatctcactatgttgcccaagctggtttcagattcctgtgctcaagggattctgctaacttggctccccaaagtgctgggattacaaatgtgagccactgtatctggcccatattcttttttaagaaaagatgcagaggtgttaaatattaatatcaaattgtccaggcatggtgtttatgaaattgtgtgccctctgacaggcaaccaaacacacacgacttcatttctttattaattcctgcctcatcatcttttctcattgatgctccttaatgtcaaaggaatctctctctctcacacacacataagaccaaaacaaatatcttgaacatgcaaaaaaatagtctacgcttttgaatagtgtgcactgttgaatagtgtgcactgttggatagtgtgcactgttgaagtgtgatgtgcctaaggcaacaggatcttgggaaagctctagatttttggcttcgaaataaaactgcatgttgaatagcaggtttttacatttattattgttgtgtatttcctcccctttttgcaatactatctacgctgagttatctattgccaactagcaccaattctccaaatcaaagtgtgtgaggaaaacacactcgtgcaatcctctttaacagaagatacaccaagtaacctgtctgtctacttctgttacccagaaataaaagaacttgaagggctgcttggctggaggggtccgggtgggagagcatcctgccctcagtcggaatccatggtgaacagctggatgtcctgtggattccagtacaggccgactgctgagttgtagacaagagaccagacataggggataaaaaactcctcgggctgctcctcttccacatatttgaatttcaattctggaaatttcagatcaatattttgcattatatcctgaaatgaaggatgagttcgaaattgttcaaagagatcgcgtttgtaaagcagggcgtataccaagtttgggttgtggtgaagggaatttgtcaggcaggagttgatgatctctaacatcattcgaatcacttcttcaatgacatttaggtcttgtgcataatctggtagaggaacatcattagaactcagcgaacctctcaaggactgtgtggcttgttccagaactttgttgtgttttttagacagcaaagaaaataaactggaagcataggatctgagaatgtgagagcaagttaaagacaagagttcctctccattgtcactgagggtcgagaagcaatgctgaagcgtagaacagtgagagtgggggaaatacagtttgtccaacacataaacatatctccgcaagtggcggcaggtataactgatgatcctctgggcagcatactgatggagagaacgaaactgtgccgacatatttgctaaagctgccaaacaatttgtgtgaaggtacttgtctcgtgtcctagtcatgttgtattgaatggttcttattaccaccaggatcaggagactccccaaggagatttcagttaaaactcgttctgaataccaagtaatattttttagtatcacttcatgaatggatctgttgaagccatcatcttccgtaaggatcaacaatattataagggccatatacacatggtgtgaattcctttcttcaacatgatacagaatctcaagaattggtaaaacaagattttccatatctgtgcgagccaacatgtatgttctaatattactattttgatggagcaaggtatacaagaggagagttgcttgatcagatgtctgctgttcacaaagagctgtgtacaaactattaaagttgatctggaaggcatgtggaattgatgaggggaaaggactgctatcttgtgtgttcttgaaggacataatggcttgtctgtaggggtttggcgcatctgaggcatctgtcagattggccaacaccagcagaagcaggagactctggttggccagaggggaagaaagctctggagaggcagccgctttgctgcccacaccacctagtgtgaagacagtccagagtcctgttgctactcctgatgcaagtccataaagcagtcctcccccatccgactgctgagggaaaacatgggcccctggaggaggtggcttttcttgtctgataaagttatataataaggtcttcacaagtttgctggtgtatggaagacatggacctcgcatcaaatacttgtggctgatgctctgtcgcaaaacttctttgtggaagagttggcaggaaaggaaaacaaccattgttgatatagcttctactgatatttcatatgtaatatctaagagtggaatatcagtgatcaactgcatcaaacagcacagcaattcttccaaaagatcttctgagtcagaactgtaattgccaggagatttttcttcataagtaaaatgaagttgtaattcctcctctgacatctgacagatgaacactttcagcaaacagcaaataataaacaaagcattgtgtgtctgccaaatgaagatgtggttctgacattctgctgaaagttttagttctttggttctagaaaggaagaccttaattagtgcaccaagatttcctgttcgaggattgttttcaactaatgacctgcagactgaaatggttgcttcctccaagagtttcaactcactactgctagttggtgcagggaaagaaaatgagagaagctgattccagaacgggtcattctcagagatagattccgtgcctgataactttttcaagtactcatttttaggaagatcgccgattctgctgctattcgatcccatcttctagcttaagcagataatttgtccttaaacctgcatttccaaaagacaacctgtctcagccggctgggggatctgctccagctccacggacccgcggacggatgggagggtggcagaggggtcaggagaagtcgctgtcgccgccgcagcccaggtggcgcacaccggctcaggcctccatgtttccacgtctcagcgggtacagatccggctccggtccggcctgcagctcggccccggctcggctccagcccgggccgcgtcggtgcggaggccaggaggcggcgagagaagaggg

SEQ ID NO: 9103 - RNA, 5863 nt, Homo sapiens
  source 1..5863: mol_type = other RNA
actggacttggagtcagaaggcctaataatcagtccctaaaatcaagtggcaactactgatattgcaggatagtgcctaggaaagaattaagagacccaaagggttgaccttgcagagactccagcctatgaagtatcagcaagtgccaaaaatttatggctctgcaaaaaagcacagggtgactcaattatgcagagagctctaccacccaatgcaaaaccctggctcccggaatctaaaggacgaaatgttgcttaaagtatgatatattaacaattccagtgcttaaaagtttccctcactaaatatttctcttggatgtaccttagcaagctcttaggaagttgctgagtgttctgatgctggtcctgtgtcctttccactttctatcgtctacttcccagctcctgtgctttccttccagagagaactgtgtgtgcagtgtactttctatgcttcaccttcagggaccttctcttctttcctttctctgtctttgtccttgagctgtgttgtctgcactgctgaatggtggcagtcctgctgcaaggttgttgttcatagattgtatgacaccagcctcaacgggtgactgtgggaactagagttagaaatctgaagctcttctgcaaagtgccttgaactcttgatagggaagatgctattgaaagggacaaattcttttaaaagtaaatattgtggcagaagtctttgttgataaaatgacacaatgcagtaacagcttcagatctggggtaaaatcagatgccaatttccatctgaacacacgatgatcctgtgttgcatcattacacatttttacttcgtgtaaaaatttctaagcaaactaatactcaaaattaatgcaagtataatgaaagtttatcattcagatttattgccatataataaatctttcacaaaaatcaggaagaagcctctggtgactttgcagagctgaggcagtgatgcacgtggtggggcctccctcctgagcgggaaccaggactgggagcatcacttgcaggcctccatggaggctgctgccccagctgagctgttagctagtgagtgcttctactgtgtgatgaatgagaaaagggaaagaggggagggcaatcagggttctgggggcacctcagtgagcccagaggcctggaggagaggctgtatgattccccagtcaggccttccttgggagtgtgccctctgtcaagatgactgggtttttgaagggcctcatttcctcacacaacaagcactgacagtcctgcagcccagggactgtcctgtggcactgcccagccctcagactcagaggacagttctgtggtcctgccagaagctcagctgttccacatgacccttaaacatttaaacaattttttggtttaaaggaaaaggaagccaatcaaaatgctttggaaacaaattaaagttgcaaattatttccccacatagtaaatacatatccttgctacctgaaatgataatcatcactccccctgctggctgagagcgcttctcctccttcagactggctctgccacaaagctaagtattagtagaagttgttgccaagcctcacctctagcctgtacatgggctctgaggtgaacacaggagtcagagtccccactccagcagtgactggaggaggcctgacagaacaagccccttggggacaggaggcaagctgcactcacctctgggaccccacccgggatgggcgctccacgagtcccttggccttagggaacctctgtttcattccatccagacgaggatagggaagcttcctgccctacctcgacagcctctaagagcacagcttggccaggccttcccgtgtggagcccacacagtggtgcactgagaggctgccagtgttttgaccttttacagagcttggggtgactgagaatggttcctccgaggccctcggaagatttgatggactcaaataacacgggcctgcagccctgggacacaggacaggagaagccagccctgacacagatgagctggcagtggattcgaacagtgtgctcagtctcgtctgggcttttgtgctttctatgttgaagaccaaatactttttctttgagaatgaaactaggctccttatctagactgtgaaggggcccgtgaggacacagagtgtgactggaaaggaaggtcccaactggccctcaatgtggccccagtggctgtttccctgcaagaagctccttcctccagctcaggcaccaacacacggatcacaccggcccagaaacaaagagcaaaacatgcttttcatcccacgtggaatacagtatgaacaaattactctcctttttctattagtgtgggtgaaggaaaaagactgttttcaaatgaagcttttctttttcccaatgattaatacagagtagattaacttaatttgtgctagactccaatttaattccagcaacagttcacaggccatattcacagaaaagttaatctgggcttcatgagaagtagccattttctttttcttttctttctttttttttttttgcgagacagggtctcactttgtggctcaggctggagtgtactggcacgttcttagctcactgcagccttgaactcctgggctcaggcaatcctcctaccttagcctcctgagtagctaggactacaggaatgtgccatcatgcctggctaatttttaagttttttgtagagatgggatctcactatgttgcccaagctggtttcagattcctgtgctcaagggattctgctaacttggctccccaaagtgctgggattacaaatgtgagccactgtatctggcccatattcttttttaagaaaagatgcagaggtgttaaatattaatatcaaattgtccaggcatggtgtttatgaaattgtgtgccctctgacaggcaaccaaacacacacgacttcatttctttattaattcctgcctcatcatcttttctcattgatgctccttaatgtcaaaggaatctctctctctcacacacacataagaccaaaacaaatatcttgaacatgcaaaaaaatagtctacgcttttgaatagtgtgcactgttgaatagtgtgcactgttggatagtgtgcactgttgaagtgtgatgtgcctaaggcaacaggatcttgggaaagctctagatttttggcttcgaaataaaactgcatgttgaatagcaggtttttacatttattattgttgtgtatttcctcccctttttgcaatactatctacgctgagttatctattgccaactagcaccaattctccaaatcaaagtgtgtgaggaaaacacactcgtgcaatcctctttaacagaagatacaccaagtaacctgtctgtctacttctgttacccagaaataaaagaacttgaagggctgcttggctggaggggtccgggtgggagagcatcctgccctcagtcggaatccatggtgaacagctggatgtcctgtggattccagtacaggccgactgctgagttgtagacaagagaccagacataggggataaaaaactcctcgggctgctcctcttccacatatttgaatttcaattctggaaatttctgacagacaagccatgaaactgtgagaacccagaagctgcatacacaaaggcctggcatgcaaggactctgtccacctgacgatcggccagcggcttcagtctgtctttgggcagcgcaacgacgccttgcttaatgatttccaggacccgttccactgacagctcagctccagcttgcagcaaccttgagctaaagaaggagatcaccagatcaatattttgcattatatcctgaaatgaaggatgagttcgaaattgttcaaagagatcgcgtttgtaaagcagggcgtataccaagtttgggttgtggtgaagggaatttgtcaggcaggagttgatgatctctaacatcattcgaatcacttcttcaatgacatttaggtcttgtgcataatctggtagaggaacatcattagaactcagcgaacctctcaaggactgtgtggcttgttccagaactttgttgtgttttttagacagcaaagaaaataaactgatgatcctctgggcagcatactgatggagagaacgaaactgtgccgacatatttgctaaagctgccaaacaatttgtgtgaaggtacttgtctcgtgtcctagtcatgttgtattgaatggttcttattaccaccaggatcaggagactccccaaggagatttcagttaaaactcgttctgaataccaagtaatattttttagtatcacttcatgaatggatctgttgaagccatcatcttccgtaaggatcaacaatattataagggccatatacacatggtgtgaattcctttcttcaacatgatacagaatctcaagaattggtaaaacaagattttccatatctgtgcgagccaacatgtatgttctaatattactattttgatggagcaaggtatacaagaggagagttgcttgatcagatgtctgctgttcacaaagagctgtgtacaaactattaaagttgatctggaaggcatgtggaattgatgaggggaaaggactgctatcttgtgtgttcttgaaggacataatggcttgtctgtaggggtttggcgcatctgaggcatctgtcagattggccaacaccagcagaagcaggagactctggttggccagaggggaagaaagctctggagaggcagccgctttgctgcccacaccacctagtgtgaagacagtccagagtcctgttgctactcctgatgcaagtccataaagcagtcctcccccatccgactgctgagggaaaacatgggcccctggaggaggtggcttttcttgtctgataaagttatataataaggtcttcacaagtttgctggtgtatggaagacatggacctcgcatcaaatacttgtggctgatgctctgtcgcaaaacttctttgtggaagagttggcaggaaaggaaaacaaccattgttgatatagcttctactgatatttcatatgtaatatctaagagtggaatatcagtgatcaactgcatcaaacagcacagcaattcttccaaaagatcttctgagtcagaactgtaattgccaggagatttttcttcataagtaaaatgaagttgtaattcctcctctgacatctgacagatgaacactttcagcaaacagcaaataataaacaaagcattgtgtgtctgccaaatgaagatgtggttctgacattctgctgaaagttttagttctttggttctagaaaggaagaccttaattagtgcaccaagatttcctgttcgaggattgttttcaactaatgacctgcagactgaaatggttgcttcctccaagagtttcaactcactactgctagttggtgcagggaaagaaaatgagagaagctgattccagaacgggtcattctcagagatagattccgtgcctgataactttttcaagtactcatttttaggaagatcgccgattctgctgctattcgatcccatcttctagcttaagcagataatttgtccttaaacctgcatttccaaaagacaacctgtctcagccggctgggggatctgctccagctccacggacccgcggacggatgggagggtggcagaggggtcaggagaagtcgctgtcgccgccgcagcccaggtggcgcacaccggctcaggcctccatgtttccacgtctcagcgggtacagatccggctccggtccggcctgcagctcggccccggctcggctccagcccgggccgcgtcggtgcggaggccaggaggcggcgagagaagaggg

SEQ ID NO: 9104 - RNA, 6028 nt, Homo sapiens
  source 1..6028: mol_type = other RNA
actggacttggagtcagaaggcctaataatcagtccctaaaatcaagtggcaactactgatattgcaggatagtgcctaggaaagaattaagagacccaaagggttgaccttgcagagactccagcctatgaagtatcagcaagtgccaaaaatttatggctctgcaaaaaagcacagggtgactcaattatgcagagagctctaccacccaatgcaaaaccctggctcccggaatctaaaggacgaaatgttgcttaaagtatgatatattaacaattccagtgcttaaaagtttccctcactaaatatttctcttggatgtaccttagcaagctcttaggaagttgctgagtgttctgatgctggtcctgtgtcctttccactttctatcgtctacttcccagctcctgtgctttccttccagagagaactgtgtgtgcagtgtactttctatgcttcaccttcagggaccttctcttctttcctttctctgtctttgtccttgagctgtgttgtctgcactgctgaatggtggcagtcctgctgcaaggttgttgttcatagattgtatgacaccagcctcaacgggtgactgtgggaactagagttagaaatctgaagctcttctgcaaagtgccttgaactcttgatagggaagatgctattgaaagggacaaattcttttaaaagtaaatattgtggcagaagtctttgttgataaaatgacacaatgcagtaacagcttcagatctggggtaaaatcagatgccaatttccatctgaacacacgatgatcctgtgttgcatcattacacatttttacttcgtgtaaaaatttctaagcaaactaatactcaaaattaatgcaagtataatgaaagtttatcattcagatttattgccatataataaatctttcacaaaaatcaggaagaagcctctggtgactttgcagagctgaggcagtgatgcacgtggtggggcctccctcctgagcgggaaccaggactgggagcatcacttgcaggcctccatggaggctgctgccccagctgagctgttagctagtgagtgcttctactgtgtgatgaatgagaaaagggaaagaggggagggcaatcagggttctgggggcacctcagtgagcccagaggcctggaggagaggctgtatgattccccagtcaggccttccttgggagtgtgccctctgtcaagatgactgggtttttgaagggcctcatttcctcacacaacaagcactgacagtcctgcagcccagggactgtcctgtggcactgcccagccctcagactcagaggacagttctgtggtcctgccagaagctcagctgttccacatgacccttaaacatttaaacaattttttggtttaaaggaaaaggaagccaatcaaaatgctttggaaacaaattaaagttgcaaattatttccccacatagtaaatacatatccttgctacctgaaatgataatcatcactccccctgctggctgagagcgcttctcctccttcagactggctctgccacaaagctaagtattagtagaagttgttgccaagcctcacctctagcctgtacatgggctctgaggtgaacacaggagtcagagtccccactccagcagtgactggaggaggcctgacagaacaagccccttggggacaggaggcaagctgcactcacctctgggaccccacccgggatgggcgctccacgagtcccttggccttagggaacctctgtttcattccatccagacgaggatagggaagcttcctgccctacctcgacagcctctaagagcacagcttggccaggccttcccgtgtggagcccacacagtggtgcactgagaggctgccagtgttttgaccttttacagagcttggggtgactgagaatggttcctccgaggccctcggaagatttgatggactcaaataacacgggcctgcagccctgggacacaggacaggagaagccagccctgacacagatgagctggcagtggattcgaacagtgtgctcagtctcgtctgggcttttgtgctttctatgttgaagaccaaatactttttctttgagaatgaaactaggctccttatctagactgtgaaggggcccgtgaggacacagagtgtgactggaaaggaaggtcccaactggccctcaatgtggccccagtggctgtttccctgcaagaagctccttcctccagctcaggcaccaacacacggatcacaccggcccagaaacaaagagcaaaacatgcttttcatcccacgtggaatacagtatgaacaaattactctcctttttctattagtgtgggtgaaggaaaaagactgttttcaaatgaagcttttctttttcccaatgattaatacagagtagattaacttaatttgtgctagactccaatttaattccagcaacagttcacaggccatattcacagaaaagttaatctgggcttcatgagaagtagccattttctttttcttttctttctttttttttttttgcgagacagggtctcactttgtggctcaggctggagtgtactggcacgttcttagctcactgcagccttgaactcctgggctcaggcaatcctcctaccttagcctcctgagtagctaggactacaggaatgtgccatcatgcctggctaatttttaagttttttgtagagatgggatctcactatgttgcccaagctggtttcagattcctgtgctcaagggattctgctaacttggctccccaaagtgctgggattacaaatgtgagccactgtatctggcccatattcttttttaagaaaagatgcagaggtgttaaatattaatatcaaattgtccaggcatggtgtttatgaaattgtgtgccctctgacaggcaaccaaacacacacgacttcatttctttattaattcctgcctcatcatcttttctcattgatgctccttaatgtcaaaggaatctctctctctcacacacacataagaccaaaacaaatatcttgaacatgcaaaaaaatagtctacgcttttgaatagtgtgcactgttgaatagtgtgcactgttggatagtgtgcactgttgaagtgtgatgtgcctaaggcaacaggatcttgggaaagctctagatttttggcttcgaaataaaactgcatgttgaatagcaggtttttacatttattattgttgtgtatttcctcccctttttgcaatactatctacgctgagttatctattgccaactagcaccaattctccaaatcaaagtgtgtgaggaaaacacactcgtgcaatcctctttaacagaagatacaccaagtaacctgtctgtctacttctgttacccagaaataaaagaacttgaagggctgcttggctggaggggtccgggtgggagagcatcctgccctcagtcggaatccatggtgaacagctggatgtcctgtggattccagtacaggccgactgctgagttgtagacaagagaccagacataggggataaaaaactcctcgggctgctcctcttccacatatttgaatttcaattctggaaatttctgacagacaagccatgaaactgtgagaacccagaagctgcatacacaaaggcctggcatgcaaggactctgtccacctgacgatcggccagcggcttcagtctgtctttgggcagcgcaacgacgccttgcttaatgatttccaggacccgttccactgacagctcagctccagcttgcagcaaccttgagctaaagaaggagatcaccagatcaatattttgcattatatcctgaaatgaaggatgagttcgaaattgttcaaagagatcgcgtttgtaaagcagggcgtataccaagtttgggttgtggtgaagggaatttgtcaggcaggagttgatgatctctaacatcattcgaatcacttcttcaatgacatttaggtcttgtgcataatctggtagaggaacatcattagaactcagcgaacctctcaaggactgtgtggcttgttccagaactttgttgtgttttttagacagcaaagaaaataaactggaagcataggatctgagaatgtgagagcaagttaaagacaagagttcctctccattgtcactgagggtcgagaagcaatgctgaagcgtagaacagtgagagtgggggaaatacagtttgtccaacacataaacatatctccgcaagtggcggcaggtataactgatgatcctctgggcagcatactgatggagagaacgaaactgtgccgacatatttgctaaagctgccaaacaatttgtgtgaaggtacttgtctcgtgtcctagtcatgttgtattgaatggttcttattaccaccaggatcaggagactccccaaggagatttcagttaaaactcgttctgaataccaagtaatattttttagtatcacttcatgaatggatctgttgaagccatcatcttccgtaaggatcaacaatattataagggccatatacacatggtgtgaattcctttcttcaacatgatacagaatctcaagaattggtaaaacaagattttccatatctgtgcgagccaacatgtatgttctaatattactattttgatggagcaaggtatacaagaggagagttgcttgatcagatgtctgctgttcacaaagagctgtgtacaaactattaaagttgatctggaaggcatgtggaattgatgaggggaaaggactgctatcttgtgtgttcttgaaggacataatggcttgtctgtaggggtttggcgcatctgaggcatctgtcagattggccaacaccagcagaagcaggagactctggttggccagaggggaagaaagctctggagaggcagccgctttgctgcccacaccacctagtgtgaagacagtccagagtcctgttgctactcctgatgcaagtccataaagcagtcctcccccatccgactgctgagggaaaacatgggcccctggaggaggtggcttttcttgtctgataaagttatataataaggtcttcacaagtttgctggtgtatggaagacatggacctcgcatcaaatacttgtggctgatgctctgtcgcaaaacttctttgtggaagagttggcaggaaaggaaaacaaccattgttgatatagcttctactgatatttcatatgtaatatctaagagtggaatatcagtgatcaactgcatcaaacagcacagcaattcttccaaaagatcttctgagtcagaactgtaattgccaggagatttttcttcataagtaaaatgaagttgtaattcctcctctgacatctgacagatgaacactttcagcaaacagcaaataataaacaaagcattgtgtgtctgccaaatgaagatgtggttctgacattctgctgaaagttttagttctttggttctagaaaggaagaccttaattagtgcaccaagatttcctgttcgaggattgttttcaactaatgacctgcagactgaaatggttgcttcctccaagagtttcaactcactactgctagttggtgcagggaaagaaaatgagagaagctgattccagaacgggtcattctcagagatagattccgtgcctgataactttttcaagtactcatttttaggaagatcgccgattctgctgctattcgatcccatcttctagcttaagcagataatttgtccttaaacctgcatttccaaaagacaacctgtctcagccggctgggggatctgctccagctccacggacccgcggacggatgggagggtggcagaggggtcaggagaagtcgctgtcgccgccgcagcccaggtggcgcacaccggctcaggcctccatgtttccacgtctcagcgggtacagatccggctccggtccggcctgcagctcggccccggctcggctccagcccgggccgcgtcggtgcggaggccaggaggcggcgagagaagaggg

SEQ ID NO: 9105 - RNA, 5015 nt, Homo sapiens
  source 1..5015: mol_type = other RNA
actggacttggagtcagaaggcctaataatcagtccctaaaatcaagtggcaactactgatattgcaggatagtgcctaggaaagaattaagagacccaaagggttgaccttgcagagactccagcctatgaagtatcagcaagtgccaaaaatttatggctctgcaaaaaagcacagggtgactcaattatgcagagagctctaccacccaatgcaaaaccctggctcccggaatctaaaggacgaaatgttgcttaaagtatgatatattaacaattccagtgcttaaaagtttccctcactaaatatttctcttggatgtaccttagcaagctcttaggaagttgctgagtgttctgatgctggtcctgtgtcctttccactttctatcgtctacttcccagctcctgtgctttccttccagagagaactgtgtgtgcagtgtactttctatgcttcaccttcagggaccttctcttctttcctttctctgtctttgtccttgagctgtgttgtctgcactgctgaatggtggcagtcctgctgcaaggttgttgttcatagattgtatgacaccagcctcaacgggtgactgtgggaactagagttagaaatctgaagctcttctgcaaagtgccttgaactcttgatagggaagatgctattgaaagggacaaattcttttaaaagtaaatattgtggcagaagtctttgttgataaaatgacacaatgcagtaacagcttcagatctggggtaaaatcagatgccaatttccatctgaacacacgatgatcctgtgttgcatcattacacatttttacttcgtgtaaaaatttctaagcaaactaatactcaaaattaatgcaagtataatgaaagtttatcattcagatttattgccatataataaatctttcacaaaaatcaggaagaagcctctggtgactttgcagagctgaggcagtgatgcacgtggtggggcctccctcctgagcgggaaccaggactgggagcatcacttgcaggcctccatggaggctgctgccccagctgagctgttagctagtgagtgcttctactgtgtgatgaatgagaaaagggaaagaggggagggcaatcagggttctgggggcacctcagtgagcccagaggcctggaggagaggctgtatgattccccagtcaggccttccttgggagtgtgccctctgtcaagatgactgggtttttgaagggcctcatttcctcacacaacaagcactgacagtcctgcagcccagggactgtcctgtggcactgcccagccctcagactcagaggacagttctgtggtcctgccagaagctcagctgttccacatgacccttaaacatttaaacaattttttggtttaaaggaaaaggaagccaatcaaaatgctttggaaacaaattaaagttgcaaattatttccccacatagtaaatacatatccttgctacctgaaatgataatcatcactccccctgctggctgagagcgcttctcctccttcagactggctctgccacaaagctaagtattagtagaagttgttgccaagcctcacctctagcctgtacatgggctctgaggtgaacacaggagtcagagtccccactccagcagtgactggaggaggcctgacagaacaagccccttggggacaggaggcaagctgcactcacctctgggaccccacccgggatgggcgctccacgagtcccttggccttagggaacctctgtttcattccatccagacgaggatagggaagcttcctgccctacctcgacagcctctaagagcacagcttggccaggccttcccgtgtggagcccacacagtggtgcactgagaggctgccagtgttttgaccttttacagagcttggggtgactgagaatggttcctccgaggccctcggaagatttgatggactcaaataacacgggcctgcagccctgggacacaggacaggagaagccagccctgacacagatgagctggcagtggattcgaacagtgtgctcagtctcgtctgggcttttgtgctttctatgttgaagaccaaatactttttctttgagaatgaaactaggctccttatctagactgtgaaggggcccgtgaggacacagagtgtgactggaaaggaaggtcccaactggccctcaatgtggccccagtggctgtttccctgcaagaagctccttcctccagctcaggcaccaacacacggatcacaccggcccagaaacaaagagcaaaacatgcttttcatcccacgtggaatacagtatgaacaaattactctcctttttctattagtgtgggtgaaggaaaaagactgttttcaaatgaagcttttctttttcccaatgattaatacagagtagattaacttaatttgtgctagactccaatttaattccagcaacagttcacaggccatattcacagaaaagttaatctgggcttcatgagaagtagccattttctttttcttttctttctttttttttttttgcgagacagggtctcactttgtggctcaggctggagtgtactggcacgttcttagctcactgcagccttgaactcctgggctcaggcaatcctcctaccttagcctcctgagtagctaggactacaggaatgtgccatcatgcctggctaatttttaagttttttgtagagatgggatctcactatgttgcccaagctggtttcagattcctgtgctcaagggattctgctaacttggctccccaaagtgctgggattacaaatgtgagccactgtatctggcccatattcttttttaagaaaagatgcagaggtgttaaatattaatatcaaattgtccaggcatggtgtttatgaaattgtgtgccctctgacaggcaaccaaacacacacgacttcatttctttattaattcctgcctcatcatcttttctcattgatgctccttaatgtcaaaggaatctctctctctcacacacacataagaccaaaacaaatatcttgaacatgcaaaaaaatagtctacgcttttgaatagtgtgcactgttgaatagtgtgcactgttggatagtgtgcactgttgaagtgtgatgtgcctaaggcaacaggatcttgggaaagctctagatttttggcttcgaaataaaactgcatgttgaatagcaggtttttacatttattattgttgtgtatttcctcccctttttgcaatactatctacgctgagttatctattgccaactagcaccaattctccaaatcaaagtgtgtgaggaaaacacactcgtgcaatcctctttaacagaagatacaccaagtaacctgtctgtctacttctgttacccagaaataaaagaacttgaagggctgcttggctggaggggtccgggtgggagagcatcctgccctcagtcggaatccatggtgaacagctggatgtcctgtggattccagtacaggccgactgctgagttgtagacaagagaccagacataggggataaaaaactcctcgggctgctcctcttccacatatttgaatttcaattctggaaatttcttcagtctgtctttgggcagcgcaacgacgccttgcttaatgatttccaggacccgttccactgacagctcagctccagcttgcagcaaccttgagctaaagaaggagatcacataatctggtagaggaacatcattagaactcagcgaacctctcaaggactgtgtggcttgttccagaactttgttgtgttttttagacagcaaagaaaataaactgatgatcctctgggcagcatactgatggagagaacgaaactgtgccgacatatttgctaaagctgccaaacaatttgtgtgaaggtacttgtctcgtgtcctagtcatgttgtattgaatggttcttattaccaccaggatcaggagactccccaaggagatttcagttaaaactcgttctgaataccaagtaatattttttagtatcacttcatgaatggatctgttgaagccatcatcttccgtaaggatcaacaatattataagggccatatacacatggtgtgaattcctttcttcaacatgatacagaatctcaagaattggtaaaacaagattttccatatctgtgcgagccaacatgtatgttctaatattactattttgatggagcaaggtatacaagaggagagttgcttgatcagatgtctgctgttcacaaagagctgtgtacaaactattaaagttgatctggaaggcatgtggaattgatgaggggaaaggactgctatcttgtgtgttcttgaaggacataatggcttgtctgtaggggtttggcgcatctgaggcatctgtcagattggccaacaccagcagaagcaggagactctggttggccagaggggaagaaagctctggagaggcagccgctttgctgcccacaccacctagtgtgaagacagtccagagtcctgctaatgacctgcagactgaaatggttgcttcctccaagagtttcaactcactactgctagttggtgcagggaaagaaaatgagagaagctgattccagaacgggtcattctcagagatagattccgtgcctgataactttttcaagtactcatttttaggaagatcgccgattctgctgctattcgatcccatcttctagcttaagcagataatttgtccttaaacctgcatttccaaaagacaacctgtctcagccggctgggggatctgctccagctccacggacccgcggacggatgggagggtggcagaggggtcaggagaagtcgctgtcgccgccgcagcccaggtggcgcacaccggctcaggcctccatgtttccacgtctcagcgggtacagatccggctccggtccggcctgcagctcggccccggctcggctccagcccgggccgcgtcggtgcggaggccaggaggcggcgagagaagaggg

SEQ ID NO: 9106 - RNA, 5585 nt, Homo sapiens
  source 1..5585: mol_type = other RNA
actggacttggagtcagaaggcctaataatcagtccctaaaatcaagtggcaactactgatattgcaggatagtgcctaggaaagaattaagagacccaaagggttgaccttgcagagactccagcctatgaagtatcagcaagtgccaaaaatttatggctctgcaaaaaagcacagggtgactcaattatgcagagagctctaccacccaatgcaaaaccctggctcccggaatctaaaggacgaaatgttgcttaaagtatgatatattaacaattccagtgcttaaaagtttccctcactaaatatttctcttggatgtaccttagcaagctcttaggaagttgctgagtgttctgatgctggtcctgtgtcctttccactttctatcgtctacttcccagctcctgtgctttccttccagagagaactgtgtgtgcagtgtactttctatgcttcaccttcagggaccttctcttctttcctttctctgtctttgtccttgagctgtgttgtctgcactgctgaatggtggcagtcctgctgcaaggttgttgttcatagattgtatgacaccagcctcaacgggtgactgtgggaactagagttagaaatctgaagctcttctgcaaagtgccttgaactcttgatagggaagatgctattgaaagggacaaattcttttaaaagtaaatattgtggcagaagtctttgttgataaaatgacacaatgcagtaacagcttcagatctggggtaaaatcagatgccaatttccatctgaacacacgatgatcctgtgttgcatcattacacatttttacttcgtgtaaaaatttctaagcaaactaatactcaaaattaatgcaagtataatgaaagtttatcattcagatttattgccatataataaatctttcacaaaaatcaggaagaagcctctggtgactttgcagagctgaggcagtgatgcacgtggtggggcctccctcctgagcgggaaccaggactgggagcatcacttgcaggcctccatggaggctgctgccccagctgagctgttagctagtgagtgcttctactgtgtgatgaatgagaaaagggaaagaggggagggcaatcagggttctgggggcacctcagtgagcccagaggcctggaggagaggctgtatgattccccagtcaggccttccttgggagtgtgccctctgtcaagatgactgggtttttgaagggcctcatttcctcacacaacaagcactgacagtcctgcagcccagggactgtcctgtggcactgcccagccctcagactcagaggacagttctgtggtcctgccagaagctcagctgttccacatgacccttaaacatttaaacaattttttggtttaaaggaaaaggaagccaatcaaaatgctttggaaacaaattaaagttgcaaattatttccccacatagtaaatacatatccttgctacctgaaatgataatcatcactccccctgctggctgagagcgcttctcctccttcagactggctctgccacaaagctaagtattagtagaagttgttgccaagcctcacctctagcctgtacatgggctctgaggtgaacacaggagtcagagtccccactccagcagtgactggaggaggcctgacagaacaagccccttggggacaggaggcaagctgcactcacctctgggaccccacccgggatgggcgctccacgagtcccttggccttagggaacctctgtttcattccatccagacgaggatagggaagcttcctgccctacctcgacagcctctaagagcacagcttggccaggccttcccgtgtggagcccacacagtggtgcactgagaggctgccagtgttttgaccttttacagagcttggggtgactgagaatggttcctccgaggccctcggaagatttgatggactcaaataacacgggcctgcagccctgggacacaggacaggagaagccagccctgacacagatgagctggcagtggattcgaacagtgtgctcagtctcgtctgggcttttgtgctttctatgttgaagaccaaatactttttctttgagaatgaaactaggctccttatctagactgtgaaggggcccgtgaggacacagagtgtgactggaaaggaaggtcccaactggccctcaatgtggccccagtggctgtttccctgcaagaagctccttcctccagctcaggcaccaacacacggatcacaccggcccagaaacaaagagcaaaacatgcttttcatcccacgtggaatacagtatgaacaaattactctcctttttctattagtgtgggtgaaggaaaaagactgttttcaaatgaagcttttctttttcccaatgattaatacagagtagattaacttaatttgtgctagactccaatttaattccagcaacagttcacaggccatattcacagaaaagttaatctgggcttcatgagaagtagccattttctttttcttttctttctttttttttttttgcgagacagggtctcactttgtggctcaggctggagtgtactggcacgttcttagctcactgcagccttgaactcctgggctcaggcaatcctcctaccttagcctcctgagtagctaggactacaggaatgtgccatcatgcctggctaatttttaagttttttgtagagatgggatctcactatgttgcccaagctggtttcagattcctgtgctcaagggattctgctaacttggctccccaaagtgctgggattacaaatgtgagccactgtatctggcccatattcttttttaagaaaagatgcagaggtgttaaatattaatatcaaattgtccaggcatggtgtttatgaaattgtgtgccctctgacaggcaaccaaacacacacgacttcatttctttattaattcctgcctcatcatcttttctcattgatgctccttaatgtcaaaggaatctctctctctcacacacacataagaccaaaacaaatatcttgaacatgcaaaaaaatagtctacgcttttgaatagtgtgcactgttgaatagtgtgcactgttggatagtgtgcactgttgaagtgtgatgtgcctaaggcaacaggatcttgggaaagctctagatttttggcttcgaaataaaactgcatgttgaatagcaggtttttacatttattattgttgtgtatttcctcccctttttgcaatactatctacgctgagttatctattgccaactagcaccaattctccaaatcaaagtgtgtgaggaaaacacactcgtgcaatcctctttaacagaagatacaccaagtaacctgtctgtctacttctgttacccagaaataaaagaacttgaagggctgcttggctggaggggtccgggtgggagagcatcctgccctcagtcggaatccatggtgaacagctggatgtcctgtggattccagtacaggccgactgctgagttgtagacaagagaccagacataggggataaaaaactcctcgggctgctcctcttccacatatttgaatttcaattctggaaatttcttcagtctgtctttgggcagcgcaacgacgccttgcttaatgatttccaggacccgttccactgacagctcagctccagcttgcagcaaccttgagctaaagaaggagatcacataatctggtagaggaacatcattagaactcagcgaacctctcaaggactgtgtggcttgttccagaactttgttgtgttttttagacagcaaagaaaataaactgatgatcctctgggcagcatactgatggagagaacgaaactgtgccgacatatttgctaaagctgccaaacaatttgtgtgaaggtacttgtctcgtgtcctagtcatgttgtattgaatggttcttattaccaccaggatcaggagactccccaaggagatttcagttaaaactcgttctgaataccaagtaatattttttagtatcacttcatgaatggatctgttgaagccatcatcttccgtaaggatcaacaatattataagggccatatacacatggtgtgaattcctttcttcaacatgatacagaatctcaagaattggtaaaacaagattttccatatctgtgcgagccaacatgtatgttctaatattactattttgatggagcaaggtatacaagaggagagttgcttgatcagatgtctgctgttcacaaagagctgtgtacaaactattaaagttgatctggaaggcatgtggaattgatgaggggaaaggactgctatcttgtgtgttcttgaaggacataatggcttgtctgtaggggtttggcgcatctgaggcatctgtcagattggccaacaccagcagaagcaggagactctggttggccagaggggaagaaagctctggagaggcagccgctttgctgcccacaccacctagtgtgaagacagtccagagtcctgttgctactcctgatgcaagtccataaagcagtcctcccccatccgactgctgagggaaaacatgggcccctggaggaggtggcttttcttgtctgataaagttatataataaggtcttcacaagtttgctggtgtatggaagacatggacctcgcatcaaatacttgtggctgatgctctgtcgcaaaacttctttgtggaagagttggcaggaaaggaaaacaaccattgttgatatagcttctactgatatttcatatgtaatatctaagagtggaatatcagtgatcaactgcatcaaacagcacagcaattcttccaaaagatcttctgagtcagaactgtaattgccaggagatttttcttcataagtaaaatgaagttgtaattcctcctctgacatctgacagatgaacactttcagcaaacagcaaataataaacaaagcattgtgtgtctgccaaatgaagatgtggttctgacattctgctgaaagttttagttctttggttctagaaaggaagaccttaattagtgcaccaagatttcctgttcgaggattgttttcaactaatgacctgcagactgaaatggttgcttcctccaagagtttcaactcactactgctagttggtgcagggaaagaaaatgagagaagctgattccagaacgggtcattctcagagatagattccgtgcctgataactttttcaagtactcatttttaggaagatcgccgattctgctgctattcgatcccatcttctagcttaagcagataatttgtccttaaacctgcatttccaaaagacaacctgtctcagccggctgggggatctgctccagctccacggacccgcggacggatgggagggtggcagaggggtcaggagaagtcgctgtcgccgccgcagcccaggtggcgcacaccggctcaggcctccatgtttccacgtctcagcgggtacagatccggctccggtccggcctgcagctcggccccggctcggctccagcccgggccgcgtcggtgcggaggccaggaggcggcgagagaagaggg

SEQ ID NO: 9107 - RNA, 5582 nt, Homo sapiens
  source 1..5582: mol_type = other RNA
actggacttggagtcagaaggcctaataatcagtccctaaaatcaagtggcaactactgatattgcaggatagtgcctaggaaagaattaagagacccaaagggttgaccttgcagagactccagcctatgaagtatcagcaagtgccaaaaatttatggctctgcaaaaaagcacagggtgactcaattatgcagagagctctaccacccaatgcaaaaccctggctcccggaatctaaaggacgaaatgttgcttaaagtatgatatattaacaattccagtgcttaaaagtttccctcactaaatatttctcttggatgtaccttagcaagctcttaggaagttgctgagtgttctgatgctggtcctgtgtcctttccactttctatcgtctacttcccagctcctgtgctttccttccagagagaactgtgtgtgcagtgtactttctatgcttcaccttcagggaccttctcttctttcctttctctgtctttgtccttgagctgtgttgtctgcactgctgaatggtggcagtcctgctgcaaggttgttgttcatagattgtatgacaccagcctcaacgggtgactgtgggaactagagttagaaatctgaagctcttctgcaaagtgccttgaactcttgatagggaagatgctattgaaagggacaaattcttttaaaagtaaatattgtggcagaagtctttgttgataaaatgacacaatgcagtaacagcttcagatctggggtaaaatcagatgccaatttccatctgaacacacgatgatcctgtgttgcatcattacacatttttacttcgtgtaaaaatttctaagcaaactaatactcaaaattaatgcaagtataatgaaagtttatcattcagatttattgccatataataaatctttcacaaaaatcaggaagaagcctctggtgactttgcagagctgaggcagtgatgcacgtggtggggcctccctcctgagcgggaaccaggactgggagcatcacttgcaggcctccatggaggctgctgccccagctgagctgttagctagtgagtgcttctactgtgtgatgaatgagaaaagggaaagaggggagggcaatcagggttctgggggcacctcagtgagcccagaggcctggaggagaggctgtatgattccccagtcaggccttccttgggagtgtgccctctgtcaagatgactgggtttttgaagggcctcatttcctcacacaacaagcactgacagtcctgcagcccagggactgtcctgtggcactgcccagccctcagactcagaggacagttctgtggtcctgccagaagctcagctgttccacatgacccttaaacatttaaacaattttttggtttaaaggaaaaggaagccaatcaaaatgctttggaaacaaattaaagttgcaaattatttccccacatagtaaatacatatccttgctacctgaaatgataatcatcactccccctgctggctgagagcgcttctcctccttcagactggctctgccacaaagctaagtattagtagaagttgttgccaagcctcacctctagcctgtacatgggctctgaggtgaacacaggagtcagagtccccactccagcagtgactggaggaggcctgacagaacaagccccttggggacaggaggcaagctgcactcacctctgggaccccacccgggatgggcgctccacgagtcccttggccttagggaacctctgtttcattccatccagacgaggatagggaagcttcctgccctacctcgacagcctctaagagcacagcttggccaggccttcccgtgtggagcccacacagtggtgcactgagaggctgccagtgttttgaccttttacagagcttggggtgactgagaatggttcctccgaggccctcggaagatttgatggactcaaataacacgggcctgcagccctgggacacaggacaggagaagccagccctgacacagatgagctggcagtggattcgaacagtgtgctcagtctcgtctgggcttttgtgctttctatgttgaagaccaaatactttttctttgagaatgaaactaggctccttatctagactgtgaaggggcccgtgaggacacagagtgtgactggaaaggaaggtcccaactggccctcaatgtggccccagtggctgtttccctgcaagaagctccttcctccagctcaggcaccaacacacggatcacaccggcccagaaacaaagagcaaaacatgcttttcatcccacgtggaatacagtatgaacaaattactctcctttttctattagtgtgggtgaaggaaaaagactgttttcaaatgaagcttttctttttcccaatgattaatacagagtagattaacttaatttgtgctagactccaatttaattccagcaacagttcacaggccatattcacagaaaagttaatctgggcttcatgagaagtagccattttctttttcttttctttctttttttttttttgcgagacagggtctcactttgtggctcaggctggagtgtactggcacgttcttagctcactgcagccttgaactcctgggctcaggcaatcctcctaccttagcctcctgagtagctaggactacaggaatgtgccatcatgcctggctaatttttaagttttttgtagagatgggatctcactatgttgcccaagctggtttcagattcctgtgctcaagggattctgctaacttggctccccaaagtgctgggattacaaatgtgagccactgtatctggcccatattcttttttaagaaaagatgcagaggtgttaaatattaatatcaaattgtccaggcatggtgtttatgaaattgtgtgccctctgacaggcaaccaaacacacacgacttcatttctttattaattcctgcctcatcatcttttctcattgatgctccttaatgtcaaaggaatctctctctctcacacacacataagaccaaaacaaatatcttgaacatgcaaaaaaatagtctacgcttttgaatagtgtgcactgttgaatagtgtgcactgttggatagtgtgcactgttgaagtgtgatgtgcctaaggcaacaggatcttgggaaagctctagatttttggcttcgaaataaaactgcatgttgaatagcaggtttttacatttattattgttgtgtatttcctcccctttttgcaatactatctacgctgagttatctattgccaactagcaccaattctccaaatcaaagtgtgtgaggaaaacacactcgtgcaatcctctttaacagaagatacaccaagtaacctgtctgtctacttctgttacccagaaataaaagaacttgaagggctgcttggctggaggggtccgggtgggagagcatcctgccctcagtcggaatccatggtgaacagctggatgtcctgtggattccagtacaggccgactgctgagttgtagacaagagaccagacataggggataaaaaactcctcgggctgctcctcttccacatatttgaatttcaattctggaaatttcttcagtctgtctttgggcagcgcaacgacgccttgcttaatgatttccaggacccgttccactgacagctcagctccagcttgcagcaaccttgagctaaagaaggagatcacataatctggtagaggaacatcattagaactcagcgaacctctcaaggactgtgtggcttgttccagaactttgttgtgttttttagacagcaaagaaaataaactgatgatcctctgggcagcatactgatggagagaacgaaactgtgccgacatatttgctaaagctgccaaacaatttgtgtgaaggtacttgtctcgtgtcctagtcatgttgtattgaatggttcttattaccaccaggatcaggagactccccaaggagatttcagttaaaactcgttctgaataccaagtaatattttttagtatcacttcatgaatggatctgttgaagccatcatcttccgtaaggatcaacaatattataagggccatatacacatggtgtgaattcctttcttcaacatgatacagaatctcaagaattggtaaaacaagattttccatatctgtgcgagccaacatgtatgttctaatattactattttgatggagcaaggtatacaagaggagagttgcttgatcagatgtctgctgttcacaaagagctgtgtacaaactattaaagttgatctggaaggcatgtggaattgatgaggggaaaggactgctatcttgtgtgttcttgaaggacataatggcttgtctgtaggggtttggcgcatctgaggcatctgtcagattggccaacaccagcagaagcaggagactctggttggccagaggggaagaaagctctggagaggcagccgctttgctgcccacaccacctagtgtgaagacagtccagagtcttgctactcctgatgcaagtccataaagcagtcctcccccatccgactgctgagggaaaacatgggcccctggaggaggtggcttttcttgtctgataaagttatataataaggtcttcacaagtttgctggtgtatggaagacatggacctcgcatcaaatacttgtggctgatgctctgtcgcaaaacttctttgtggaagagttggcaggaaaggaaaacaaccattgttgatatagcttctactgatatttcatatgtaatatctaagagtggaatatcagtgatcaactgcatcaaacagcacagcaattcttccaaaagatcttctgagtcagaactgtaattgccaggagatttttcttcataagtaaaatgaagttgtaattcctcctctgacatctgacagatgaacactttcagcaaacagcaaataataaacaaagcattgtgtgtctgccaaatgaagatgtggttctgacattctgctgaaagttttagttctttggttctagaaaggaagaccttaattagtgcaccaagatttcctgttcgaggattgttttcaactaatgacctgcagactgaaatggttgcttcctccaagagtttcaactcactactgctagttggtgcagggaaagaaaatgagagaagctgattccagaacgggtcattctcagagatagattccgtgcctgataactttttcaagtactcatttttaggaagatcgccgattctgctgctattcgatcccatcttctagcttaagcagataatttgtccttaaacctgcatttccaaaagacaacctgtctcagccggctgggggatctgctccagctccacggacccgcggacggatgggagggtggcagaggggtcaggagaagtcgctgtcgccgccgcagcccaggtggcgcacaccggctcaggcctccatgtttccacgtctcagcgggtacagatccggctccggtccggcctgcagctcggccccggctcggctccagcccgggccgcgtcggtgcggaggccaggaggcggcgagagaagaggg

SEQ ID NO: 9108 - RNA, 5579 nt, Homo sapiens
  source 1..5579: mol_type = other RNA
actggacttggagtcagaaggcctaataatcagtccctaaaatcaagtggcaactactgatattgcaggatagtgcctaggaaagaattaagagacccaaagggttgaccttgcagagactccagcctatgaagtatcagcaagtgccaaaaatttatggctctgcaaaaaagcacagggtgactcaattatgcagagagctctaccacccaatgcaaaaccctggctcccggaatctaaaggacgaaatgttgcttaaagtatgatatattaacaattccagtgcttaaaagtttccctcactaaatatttctcttggatgtaccttagcaagctcttaggaagttgctgagtgttctgatgctggtcctgtgtcctttccactttctatcgtctacttcccagctcctgtgctttccttccagagagaactgtgtgtgcagtgtactttctatgcttcaccttcagggaccttctcttctttcctttctctgtctttgtccttgagctgtgttgtctgcactgctgaatggtggcagtcctgctgcaaggttgttgttcatagattgtatgacaccagcctcaacgggtgactgtgggaactagagttagaaatctgaagctcttctgcaaagtgccttgaactcttgatagggaagatgctattgaaagggacaaattcttttaaaagtaaatattgtggcagaagtctttgttgataaaatgacacaatgcagtaacagcttcagatctggggtaaaatcagatgccaatttccatctgaacacacgatgatcctgtgttgcatcattacacatttttacttcgtgtaaaaatttctaagcaaactaatactcaaaattaatgcaagtataatgaaagtttatcattcagatttattgccatataataaatctttcacaaaaatcaggaagaagcctctggtgactttgcagagctgaggcagtgatgcacgtggtggggcctccctcctgagcgggaaccaggactgggagcatcacttgcaggcctccatggaggctgctgccccagctgagctgttagctagtgagtgcttctactgtgtgatgaatgagaaaagggaaagaggggagggcaatcagggttctgggggcacctcagtgagcccagaggcctggaggagaggctgtatgattccccagtcaggccttccttgggagtgtgccctctgtcaagatgactgggtttttgaagggcctcatttcctcacacaacaagcactgacagtcctgcagcccagggactgtcctgtggcactgcccagccctcagactcagaggacagttctgtggtcctgccagaagctcagctgttccacatgacccttaaacatttaaacaattttttggtttaaaggaaaaggaagccaatcaaaatgctttggaaacaaattaaagttgcaaattatttccccacatagtaaatacatatccttgctacctgaaatgataatcatcactccccctgctggctgagagcgcttctcctccttcagactggctctgccacaaagctaagtattagtagaagttgttgccaagcctcacctctagcctgtacatgggctctgaggtgaacacaggagtcagagtccccactccagcagtgactggaggaggcctgacagaacaagccccttggggacaggaggcaagctgcactcacctctgggaccccacccgggatgggcgctccacgagtcccttggccttagggaacctctgtttcattccatccagacgaggatagggaagcttcctgccctacctcgacagcctctaagagcacagcttggccaggccttcccgtgtggagcccacacagtggtgcactgagaggctgccagtgttttgaccttttacagagcttggggtgactgagaatggttcctccgaggccctcggaagatttgatggactcaaataacacgggcctgcagccctgggacacaggacaggagaagccagccctgacacagatgagctggcagtggattcgaacagtgtgctcagtctcgtctgggcttttgtgctttctatgttgaagaccaaatactttttctttgagaatgaaactaggctccttatctagactgtgaaggggcccgtgaggacacagagtgtgactggaaaggaaggtcccaactggccctcaatgtggccccagtggctgtttccctgcaagaagctccttcctccagctcaggcaccaacacacggatcacaccggcccagaaacaaagagcaaaacatgcttttcatcccacgtggaatacagtatgaacaaattactctcctttttctattagtgtgggtgaaggaaaaagactgttttcaaatgaagcttttctttttcccaatgattaatacagagtagattaacttaatttgtgctagactccaatttaattccagcaacagttcacaggccatattcacagaaaagttaatctgggcttcatgagaagtagccattttctttttcttttctttctttttttttttttgcgagacagggtctcactttgtggctcaggctggagtgtactggcacgttcttagctcactgcagccttgaactcctgggctcaggcaatcctcctaccttagcctcctgagtagctaggactacaggaatgtgccatcatgcctggctaatttttaagttttttgtagagatgggatctcactatgttgcccaagctggtttcagattcctgtgctcaagggattctgctaacttggctccccaaagtgctgggattacaaatgtgagccactgtatctggcccatattcttttttaagaaaagatgcagaggtgttaaatattaatatcaaattgtccaggcatggtgtttatgaaattgtgtgccctctgacaggcaaccaaacacacacgacttcatttctttattaattcctgcctcatcatcttttctcattgatgctccttaatgtcaaaggaatctctctctctcacacacacataagaccaaaacaaatatcttgaacatgcaaaaaaatagtctacgcttttgaatagtgtgcactgttgaatagtgtgcactgttggatagtgtgcactgttgaagtgtgatgtgcctaaggcaacaggatcttgggaaagctctagatttttggcttcgaaataaaactgcatgttgaatagcaggtttttacatttattattgttgtgtatttcctcccctttttgcaatactatctacgctgagttatctattgccaactagcaccaattctccaaatcaaagtgtgtgaggaaaacacactcgtgcaatcctctttaacagaagatacaccaagtaacctgtctgtctacttctgttacccagaaataaaagaacttgaagggctgcttggctggaggggtccgggtgggagagcatcctgccctcagtcggaatccatggtgaacagctggatgtcctgtggattccagtacaggccgactgctgagttgtagacaagagaccagacataggggataaaaaactcctcgggctgctcctcttccacatatttgaatttcaattctggaaatttcttcagtctgtctttgggcagcgcaacgacgccttgcttaatgatttccaggacccgttccactgacagctcagctccagcttgcagcaaccttgagctaaagaaggagatcacataatctggtagaggaacatcattagaactcagcgaacctctcaaggactgtgtggcttgttccagaactttgttgtgttttttagacagcaaagaaaataaactgatgatcctctgggcagcatactgatggagagaacgaaactgtgccgacatatttgctaaagctgccaaacaatttgtgtgaaggtacttgtctcgtgtcctagtcatgttgtattgaatggttcttattaccaccaggatcaggagactccccaaggagatttcagttaaaactcgttctgaataccaagtaatattttttagtatcacttcatgaatggatctgttgaagccatcatcttccgtaaggatcaacaatattataagggccatatacacatggtgtgaattcctttcttcaacatgatacagaatctcaagaattggtaaaacaagattttccatatctgtgcgagccaacatgtatgttctaatattactattttgatggagcaaggtatacaagaggagagttgcttgatcagatgtctgctgttcacaaagagctgtgtacaaactattaaagttgatctggaaggcatgtggaattgatgaggggaaaggactgctatcttgtgtgttcttgaaggacataatggcttgtctgtaggggtttggcgcatctgaggcatctgtcagattggccaacaccagcagaagcaggagactctggttggccagaggggaagaaagctctggagaggcagccgctttgctgcccacaccacctagtgtgaagacagtccagagtcttgctactcctgatgcaagtccataaagcagtcctcccccatccgactgctgagggaaaacatgggcccctggaggaggtggcttttcttgtctgataaagttatataataaggtcttcacaagtttgctggtgtatggaagacatggacctcgcatcaaatacttgtggctgatgctctgtcgcaaaacttctttgtggaagagttggcaggaaaggaaaacaaccattgttgatatagcttctactgatatttcatatgtaatatctaagagtggaatatcagtgatcaactgcatcaaacagcacagcaattcttccaaaagatcttctgagtcagaactgtaattgccaggagatttttcttcataagtaaaatgaagttgtaattcctcctctgacatctgacagatgaacactttcagcaaacagcaaataataaacaaagcattgtgtgtctgccaaatgaagatgtggttctgacattctgctgaaagttttagttctttggttctagaaaggaagaccttaattagtgcaccaagatttcctgttcgaggattgttttcaactaatgacctgcagactgaaatggttgcttcctccaagagtttcaactcactgctagttggtgcagggaaagaaaatgagagaagctgattccagaacgggtcattctcagagatagattccgtgcctgataactttttcaagtactcatttttaggaagatcgccgattctgctgctattcgatcccatcttctagcttaagcagataatttgtccttaaacctgcatttccaaaagacaacctgtctcagccggctgggggatctgctccagctccacggacccgcggacggatgggagggtggcagaggggtcaggagaagtcgctgtcgccgccgcagcccaggtggcgcacaccggctcaggcctccatgtttccacgtctcagcgggtacagatccggctccggtccggcctgcagctcggccccggctcggctccagcccgggccgcgtcggtgcggaggccaggaggcggcgagagaagaggg

SEQ ID NO: 9109 - RNA, 5750 nt, Homo sapiens
  source 1..5750: mol_type = other RNA
actggacttggagtcagaaggcctaataatcagtccctaaaatcaagtggcaactactgatattgcaggatagtgcctaggaaagaattaagagacccaaagggttgaccttgcagagactccagcctatgaagtatcagcaagtgccaaaaatttatggctctgcaaaaaagcacagggtgactcaattatgcagagagctctaccacccaatgcaaaaccctggctcccggaatctaaaggacgaaatgttgcttaaagtatgatatattaacaattccagtgcttaaaagtttccctcactaaatatttctcttggatgtaccttagcaagctcttaggaagttgctgagtgttctgatgctggtcctgtgtcctttccactttctatcgtctacttcccagctcctgtgctttccttccagagagaactgtgtgtgcagtgtactttctatgcttcaccttcagggaccttctcttctttcctttctctgtctttgtccttgagctgtgttgtctgcactgctgaatggtggcagtcctgctgcaaggttgttgttcatagattgtatgacaccagcctcaacgggtgactgtgggaactagagttagaaatctgaagctcttctgcaaagtgccttgaactcttgatagggaagatgctattgaaagggacaaattcttttaaaagtaaatattgtggcagaagtctttgttgataaaatgacacaatgcagtaacagcttcagatctggggtaaaatcagatgccaatttccatctgaacacacgatgatcctgtgttgcatcattacacatttttacttcgtgtaaaaatttctaagcaaactaatactcaaaattaatgcaagtataatgaaagtttatcattcagatttattgccatataataaatctttcacaaaaatcaggaagaagcctctggtgactttgcagagctgaggcagtgatgcacgtggtggggcctccctcctgagcgggaaccaggactgggagcatcacttgcaggcctccatggaggctgctgccccagctgagctgttagctagtgagtgcttctactgtgtgatgaatgagaaaagggaaagaggggagggcaatcagggttctgggggcacctcagtgagcccagaggcctggaggagaggctgtatgattccccagtcaggccttccttgggagtgtgccctctgtcaagatgactgggtttttgaagggcctcatttcctcacacaacaagcactgacagtcctgcagcccagggactgtcctgtggcactgcccagccctcagactcagaggacagttctgtggtcctgccagaagctcagctgttccacatgacccttaaacatttaaacaattttttggtttaaaggaaaaggaagccaatcaaaatgctttggaaacaaattaaagttgcaaattatttccccacatagtaaatacatatccttgctacctgaaatgataatcatcactccccctgctggctgagagcgcttctcctccttcagactggctctgccacaaagctaagtattagtagaagttgttgccaagcctcacctctagcctgtacatgggctctgaggtgaacacaggagtcagagtccccactccagcagtgactggaggaggcctgacagaacaagccccttggggacaggaggcaagctgcactcacctctgggaccccacccgggatgggcgctccacgagtcccttggccttagggaacctctgtttcattccatccagacgaggatagggaagcttcctgccctacctcgacagcctctaagagcacagcttggccaggccttcccgtgtggagcccacacagtggtgcactgagaggctgccagtgttttgaccttttacagagcttggggtgactgagaatggttcctccgaggccctcggaagatttgatggactcaaataacacgggcctgcagccctgggacacaggacaggagaagccagccctgacacagatgagctggcagtggattcgaacagtgtgctcagtctcgtctgggcttttgtgctttctatgttgaagaccaaatactttttctttgagaatgaaactaggctccttatctagactgtgaaggggcccgtgaggacacagagtgtgactggaaaggaaggtcccaactggccctcaatgtggccccagtggctgtttccctgcaagaagctccttcctccagctcaggcaccaacacacggatcacaccggcccagaaacaaagagcaaaacatgcttttcatcccacgtggaatacagtatgaacaaattactctcctttttctattagtgtgggtgaaggaaaaagactgttttcaaatgaagcttttctttttcccaatgattaatacagagtagattaacttaatttgtgctagactccaatttaattccagcaacagttcacaggccatattcacagaaaagttaatctgggcttcatgagaagtagccattttctttttcttttctttctttttttttttttgcgagacagggtctcactttgtggctcaggctggagtgtactggcacgttcttagctcactgcagccttgaactcctgggctcaggcaatcctcctaccttagcctcctgagtagctaggactacaggaatgtgccatcatgcctggctaatttttaagttttttgtagagatgggatctcactatgttgcccaagctggtttcagattcctgtgctcaagggattctgctaacttggctccccaaagtgctgggattacaaatgtgagccactgtatctggcccatattcttttttaagaaaagatgcagaggtgttaaatattaatatcaaattgtccaggcatggtgtttatgaaattgtgtgccctctgacaggcaaccaaacacacacgacttcatttctttattaattcctgcctcatcatcttttctcattgatgctccttaatgtcaaaggaatctctctctctcacacacacataagaccaaaacaaatatcttgaacatgcaaaaaaatagtctacgcttttgaatagtgtgcactgttgaatagtgtgcactgttggatagtgtgcactgttgaagtgtgatgtgcctaaggcaacaggatcttgggaaagctctagatttttggcttcgaaataaaactgcatgttgaatagcaggtttttacatttattattgttgtgtatttcctcccctttttgcaatactatctacgctgagttatctattgccaactagcaccaattctccaaatcaaagtgtgtgaggaaaacacactcgtgcaatcctctttaacagaagatacaccaagtaacctgtctgtctacttctgttacccagaaataaaagaacttgaagggctgcttggctggaggggtccgggtgggagagcatcctgccctcagtcggaatccatggtgaacagctggatgtcctgtggattccagtacaggccgactgctgagttgtagacaagagaccagacataggggataaaaaactcctcgggctgctcctcttccacatatttgaatttcaattctggaaatttcttcagtctgtctttgggcagcgcaacgacgccttgcttaatgatttccaggacccgttccactgacagctcagctccagcttgcagcaaccttgagctaaagaaggagatcacataatctggtagaggaacatcattagaactcagcgaacctctcaaggactgtgtggcttgttccagaactttgttgtgttttttagacagcaaagaaaataaactggaagcataggatctgagaatgtgagagcaagttaaagacaagagttcctctccattgtcactgagggtcgagaagcaatgctgaagcgtagaacagtgagagtgggggaaatacagtttgtccaacacataaacatatctccgcaagtggcggcaggtataactgatgatcctctgggcagcatactgatggagagaacgaaactgtgccgacatatttgctaaagctgccaaacaatttgtgtgaaggtacttgtctcgtgtcctagtcatgttgtattgaatggttcttattaccaccaggatcaggagactccccaaggagatttcagttaaaactcgttctgaataccaagtaatattttttagtatcacttcatgaatggatctgttgaagccatcatcttccgtaaggatcaacaatattataagggccatatacacatggtgtgaattcctttcttcaacatgatacagaatctcaagaattggtaaaacaagattttccatatctgtgcgagccaacatgtatgttctaatattactattttgatggagcaaggtatacaagaggagagttgcttgatcagatgtctgctgttcacaaagagctgtgtacaaactattaaagttgatctggaaggcatgtggaattgatgaggggaaaggactgctatcttgtgtgttcttgaaggacataatggcttgtctgtaggggtttggcgcatctgaggcatctgtcagattggccaacaccagcagaagcaggagactctggttggccagaggggaagaaagctctggagaggcagccgctttgctgcccacaccacctagtgtgaagacagtccagagtcctgttgctactcctgatgcaagtccataaagcagtcctcccccatccgactgctgagggaaaacatgggcccctggaggaggtggcttttcttgtctgataaagttatataataaggtcttcacaagtttgctggtgtatggaagacatggacctcgcatcaaatacttgtggctgatgctctgtcgcaaaacttctttgtggaagagttggcaggaaaggaaaacaaccattgttgatatagcttctactgatatttcatatgtaatatctaagagtggaatatcagtgatcaactgcatcaaacagcacagcaattcttccaaaagatcttctgagtcagaactgtaattgccaggagatttttcttcataagtaaaatgaagttgtaattcctcctctgacatctgacagatgaacactttcagcaaacagcaaataataaacaaagcattgtgtgtctgccaaatgaagatgtggttctgacattctgctgaaagttttagttctttggttctagaaaggaagaccttaattagtgcaccaagatttcctgttcgaggattgttttcaactaatgacctgcagactgaaatggttgcttcctccaagagtttcaactcactactgctagttggtgcagggaaagaaaatgagagaagctgattccagaacgggtcattctcagagatagattccgtgcctgataactttttcaagtactcatttttaggaagatcgccgattctgctgctattcgatcccatcttctagcttaagcagataatttgtccttaaacctgcatttccaaaagacaacctgtctcagccggctgggggatctgctccagctccacggacccgcggacggatgggagggtggcagaggggtcaggagaagtcgctgtcgccgccgcagcccaggtggcgcacaccggctcaggcctccatgtttccacgtctcagcgggtacagatccggctccggtccggcctgcagctcggccccggctcggctccagcccgggccgcgtcggtgcggaggccaggaggcggcgagagaagaggg

SEQ ID NO: 9110 - RNA, 5195 nt, Homo sapiens
  source 1..5195: mol_type = other RNA
actggacttggagtcagaaggcctaataatcagtccctaaaatcaagtggcaactactgatattgcaggatagtgcctaggaaagaattaagagacccaaagggttgaccttgcagagactccagcctatgaagtatcagcaagtgccaaaaatttatggctctgcaaaaaagcacagggtgactcaattatgcagagagctctaccacccaatgcaaaaccctggctcccggaatctaaaggacgaaatgttgcttaaagtatgatatattaacaattccagtgcttaaaagtttccctcactaaatatttctcttggatgtaccttagcaagctcttaggaagttgctgagtgttctgatgctggtcctgtgtcctttccactttctatcgtctacttcccagctcctgtgctttccttccagagagaactgtgtgtgcagtgtactttctatgcttcaccttcagggaccttctcttctttcctttctctgtctttgtccttgagctgtgttgtctgcactgctgaatggtggcagtcctgctgcaaggttgttgttcatagattgtatgacaccagcctcaacgggtgactgtgggaactagagttagaaatctgaagctcttctgcaaagtgccttgaactcttgatagggaagatgctattgaaagggacaaattcttttaaaagtaaatattgtggcagaagtctttgttgataaaatgacacaatgcagtaacagcttcagatctggggtaaaatcagatgccaatttccatctgaacacacgatgatcctgtgttgcatcattacacatttttacttcgtgtaaaaatttctaagcaaactaatactcaaaattaatgcaagtataatgaaagtttatcattcagatttattgccatataataaatctttcacaaaaatcaggaagaagcctctggtgactttgcagagctgaggcagtgatgcacgtggtggggcctccctcctgagcgggaaccaggactgggagcatcacttgcaggcctccatggaggctgctgccccagctgagctgttagctagtgagtgcttctactgtgtgatgaatgagaaaagggaaagaggggagggcaatcagggttctgggggcacctcagtgagcccagaggcctggaggagaggctgtatgattccccagtcaggccttccttgggagtgtgccctctgtcaagatgactgggtttttgaagggcctcatttcctcacacaacaagcactgacagtcctgcagcccagggactgtcctgtggcactgcccagccctcagactcagaggacagttctgtggtcctgccagaagctcagctgttccacatgacccttaaacatttaaacaattttttggtttaaaggaaaaggaagccaatcaaaatgctttggaaacaaattaaagttgcaaattatttccccacatagtaaatacatatccttgctacctgaaatgataatcatcactccccctgctggctgagagcgcttctcctccttcagactggctctgccacaaagctaagtattagtagaagttgttgccaagcctcacctctagcctgtacatgggctctgaggtgaacacaggagtcagagtccccactccagcagtgactggaggaggcctgacagaacaagccccttggggacaggaggcaagctgcactcacctctgggaccccacccgggatgggcgctccacgagtcccttggccttagggaacctctgtttcattccatccagacgaggatagggaagcttcctgccctacctcgacagcctctaagagcacagcttggccaggccttcccgtgtggagcccacacagtggtgcactgagaggctgccagtgttttgaccttttacagagcttggggtgactgagaatggttcctccgaggccctcggaagatttgatggactcaaataacacgggcctgcagccctgggacacaggacaggagaagccagccctgacacagatgagctggcagtggattcgaacagtgtgctcagtctcgtctgggcttttgtgctttctatgttgaagaccaaatactttttctttgagaatgaaactaggctccttatctagactgtgaaggggcccgtgaggacacagagtgtgactggaaaggaaggtcccaactggccctcaatgtggccccagtggctgtttccctgcaagaagctccttcctccagctcaggcaccaacacacggatcacaccggcccagaaacaaagagcaaaacatgcttttcatcccacgtggaatacagtatgaacaaattactctcctttttctattagtgtgggtgaaggaaaaagactgttttcaaatgaagcttttctttttcccaatgattaatacagagtagattaacttaatttgtgctagactccaatttaattccagcaacagttcacaggccatattcacagaaaagttaatctgggcttcatgagaagtagccattttctttttcttttctttctttttttttttttgcgagacagggtctcactttgtggctcaggctggagtgtactggcacgttcttagctcactgcagccttgaactcctgggctcaggcaatcctcctaccttagcctcctgagtagctaggactacaggaatgtgccatcatgcctggctaatttttaagttttttgtagagatgggatctcactatgttgcccaagctggtttcagattcctgtgctcaagggattctgctaacttggctccccaaagtgctgggattacaaatgtgagccactgtatctggcccatattcttttttaagaaaagatgcagaggtgttaaatattaatatcaaattgtccaggcatggtgtttatgaaattgtgtgccctctgacaggcaaccaaacacacacgacttcatttctttattaattcctgcctcatcatcttttctcattgatgctccttaatgtcaaaggaatctctctctctcacacacacataagaccaaaacaaatatcttgaacatgcaaaaaaatagtctacgcttttgaatagtgtgcactgttgaatagtgtgcactgttggatagtgtgcactgttgaagtgtgatgtgcctaaggcaacaggatcttgggaaagctctagatttttggcttcgaaataaaactgcatgttgaatagcaggtttttacatttattattgttgtgtatttcctcccctttttgcaatactatctacgctgagttatctattgccaactagcaccaattctccaaatcaaagtgtgtgaggaaaacacactcgtgcaatcctctttaacagaagatacaccaagtaacctgtctgtctacttctgttacccagaaataaaagaacttgaagggctgcttggctggaggggtccgggtgggagagcatcctgccctcagtcggaatccatggtgaacagctggatgtcctgtggattccagtacaggccgactgctgagttgtagacaagagaccagacataggggataaaaaactcctcgggctgctcctcttccacatatttgaatttcaattctggaaatttcttcagtctgtctttgggcagcgcaacgacgccttgcttaatgatttccaggacccgttccactgacagctcagctccagcttgcagcaaccttgagctaaagaaggagatcaccagatcaatattttgcattatatcctgaaatgaaggatgagttcgaaattgttcaaagagatcgcgtttgtaaagcagggcgtataccaagtttgggttgtggtgaagggaatttgtcaggcaggagttgatgatctctaacatcattcgaatcacttcttcaatgacatttaggtcttgtgcataatctggtagaggaacatcattagaactcagcgaacctctcaaggactgtgtggcttgttccagaactttgttgtgttttttagacagcaaagaaaataaactgatgatcctctgggcagcatactgatggagagaacgaaactgtgccgacatatttgctaaagctgccaaacaatttgtgtgaaggtacttgtctcgtgtcctagtcatgttgtattgaatggttcttattaccaccaggatcaggagactccccaaggagatttcagttaaaactcgttctgaataccaagtaatattttttagtatcacttcatgaatggatctgttgaagccatcatcttccgtaaggatcaacaatattataagggccatatacacatggtgtgaattcctttcttcaacatgatacagaatctcaagaattggtaaaacaagattttccatatctgtgcgagccaacatgtatgttctaatattactattttgatggagcaaggtatacaagaggagagttgcttgatcagatgtctgctgttcacaaagagctgtgtacaaactattaaagttgatctggaaggcatgtggaattgatgaggggaaaggactgctatcttgtgtgttcttgaaggacataatggcttgtctgtaggggtttggcgcatctgaggcatctgtcagattggccaacaccagcagaagcaggagactctggttggccagaggggaagaaagctctggagaggcagccgctttgctgcccacaccacctagtgtgaagacagtccagagtcctaatgacctgcagactgaaatggttgcttcctccaagagtttcaactcactactgctagttggtgcagggaaagaaaatgagagaagctgattccagaacgggtcattctcagagatagattccgtgcctgataactttttcaagtactcatttttaggaagatcgccgattctgctgctattcgatcccatcttctagcttaagcagataatttgtccttaaacctgcatttccaaaagacaacctgtctcagccggctgggggatctgctccagctccacggacccgcggacggatgggagggtggcagaggggtcaggagaagtcgctgtcgccgccgcagcccaggtggcgcacaccggctcaggcctccatgtttccacgtctcagcgggtacagatccggctccggtccggcctgcagctcggccccggctcggctccagcccgggccgcgtcggtgcggaggccaggaggcggcgagagaagaggg

SEQ ID NO: 9111 - RNA, 5198 nt, Homo sapiens
  source 1..5198: mol_type = other RNA
actggacttggagtcagaaggcctaataatcagtccctaaaatcaagtggcaactactgatattgcaggatagtgcctaggaaagaattaagagacccaaagggttgaccttgcagagactccagcctatgaagtatcagcaagtgccaaaaatttatggctctgcaaaaaagcacagggtgactcaattatgcagagagctctaccacccaatgcaaaaccctggctcccggaatctaaaggacgaaatgttgcttaaagtatgatatattaacaattccagtgcttaaaagtttccctcactaaatatttctcttggatgtaccttagcaagctcttaggaagttgctgagtgttctgatgctggtcctgtgtcctttccactttctatcgtctacttcccagctcctgtgctttccttccagagagaactgtgtgtgcagtgtactttctatgcttcaccttcagggaccttctcttctttcctttctctgtctttgtccttgagctgtgttgtctgcactgctgaatggtggcagtcctgctgcaaggttgttgttcatagattgtatgacaccagcctcaacgggtgactgtgggaactagagttagaaatctgaagctcttctgcaaagtgccttgaactcttgatagggaagatgctattgaaagggacaaattcttttaaaagtaaatattgtggcagaagtctttgttgataaaatgacacaatgcagtaacagcttcagatctggggtaaaatcagatgccaatttccatctgaacacacgatgatcctgtgttgcatcattacacatttttacttcgtgtaaaaatttctaagcaaactaatactcaaaattaatgcaagtataatgaaagtttatcattcagatttattgccatataataaatctttcacaaaaatcaggaagaagcctctggtgactttgcagagctgaggcagtgatgcacgtggtggggcctccctcctgagcgggaaccaggactgggagcatcacttgcaggcctccatggaggctgctgccccagctgagctgttagctagtgagtgcttctactgtgtgatgaatgagaaaagggaaagaggggagggcaatcagggttctgggggcacctcagtgagcccagaggcctggaggagaggctgtatgattccccagtcaggccttccttgggagtgtgccctctgtcaagatgactgggtttttgaagggcctcatttcctcacacaacaagcactgacagtcctgcagcccagggactgtcctgtggcactgcccagccctcagactcagaggacagttctgtggtcctgccagaagctcagctgttccacatgacccttaaacatttaaacaattttttggtttaaaggaaaaggaagccaatcaaaatgctttggaaacaaattaaagttgcaaattatttccccacatagtaaatacatatccttgctacctgaaatgataatcatcactccccctgctggctgagagcgcttctcctccttcagactggctctgccacaaagctaagtattagtagaagttgttgccaagcctcacctctagcctgtacatgggctctgaggtgaacacaggagtcagagtccccactccagcagtgactggaggaggcctgacagaacaagccccttggggacaggaggcaagctgcactcacctctgggaccccacccgggatgggcgctccacgagtcccttggccttagggaacctctgtttcattccatccagacgaggatagggaagcttcctgccctacctcgacagcctctaagagcacagcttggccaggccttcccgtgtggagcccacacagtggtgcactgagaggctgccagtgttttgaccttttacagagcttggggtgactgagaatggttcctccgaggccctcggaagatttgatggactcaaataacacgggcctgcagccctgggacacaggacaggagaagccagccctgacacagatgagctggcagtggattcgaacagtgtgctcagtctcgtctgggcttttgtgctttctatgttgaagaccaaatactttttctttgagaatgaaactaggctccttatctagactgtgaaggggcccgtgaggacacagagtgtgactggaaaggaaggtcccaactggccctcaatgtggccccagtggctgtttccctgcaagaagctccttcctccagctcaggcaccaacacacggatcacaccggcccagaaacaaagagcaaaacatgcttttcatcccacgtggaatacagtatgaacaaattactctcctttttctattagtgtgggtgaaggaaaaagactgttttcaaatgaagcttttctttttcccaatgattaatacagagtagattaacttaatttgtgctagactccaatttaattccagcaacagttcacaggccatattcacagaaaagttaatctgggcttcatgagaagtagccattttctttttcttttctttctttttttttttttgcgagacagggtctcactttgtggctcaggctggagtgtactggcacgttcttagctcactgcagccttgaactcctgggctcaggcaatcctcctaccttagcctcctgagtagctaggactacaggaatgtgccatcatgcctggctaatttttaagttttttgtagagatgggatctcactatgttgcccaagctggtttcagattcctgtgctcaagggattctgctaacttggctccccaaagtgctgggattacaaatgtgagccactgtatctggcccatattcttttttaagaaaagatgcagaggtgttaaatattaatatcaaattgtccaggcatggtgtttatgaaattgtgtgccctctgacaggcaaccaaacacacacgacttcatttctttattaattcctgcctcatcatcttttctcattgatgctccttaatgtcaaaggaatctctctctctcacacacacataagaccaaaacaaatatcttgaacatgcaaaaaaatagtctacgcttttgaatagtgtgcactgttgaatagtgtgcactgttggatagtgtgcactgttgaagtgtgatgtgcctaaggcaacaggatcttgggaaagctctagatttttggcttcgaaataaaactgcatgttgaatagcaggtttttacatttattattgttgtgtatttcctcccctttttgcaatactatctacgctgagttatctattgccaactagcaccaattctccaaatcaaagtgtgtgaggaaaacacactcgtgcaatcctctttaacagaagatacaccaagtaacctgtctgtctacttctgttacccagaaataaaagaacttgaagggctgcttggctggaggggtccgggtgggagagcatcctgccctcagtcggaatccatggtgaacagctggatgtcctgtggattccagtacaggccgactgctgagttgtagacaagagaccagacataggggataaaaaactcctcgggctgctcctcttccacatatttgaatttcaattctggaaatttcttcagtctgtctttgggcagcgcaacgacgccttgcttaatgatttccaggacccgttccactgacagctcagctccagcttgcagcaaccttgagctaaagaaggagatcaccagatcaatattttgcattatatcctgaaatgaaggatgagttcgaaattgttcaaagagatcgcgtttgtaaagcagggcgtataccaagtttgggttgtggtgaagggaatttgtcaggcaggagttgatgatctctaacatcattcgaatcacttcttcaatgacatttaggtcttgtgcataatctggtagaggaacatcattagaactcagcgaacctctcaaggactgtgtggcttgttccagaactttgttgtgttttttagacagcaaagaaaataaactgatgatcctctgggcagcatactgatggagagaacgaaactgtgccgacatatttgctaaagctgccaaacaatttgtgtgaaggtacttgtctcgtgtcctagtcatgttgtattgaatggttcttattaccaccaggatcaggagactccccaaggagatttcagttaaaactcgttctgaataccaagtaatattttttagtatcacttcatgaatggatctgttgaagccatcatcttccgtaaggatcaacaatattataagggccatatacacatggtgtgaattcctttcttcaacatgatacagaatctcaagaattggtaaaacaagattttccatatctgtgcgagccaacatgtatgttctaatattactattttgatggagcaaggtatacaagaggagagttgcttgatcagatgtctgctgttcacaaagagctgtgtacaaactattaaagttgatctggaaggcatgtggaattgatgaggggaaaggactgctatcttgtgtgttcttgaaggacataatggcttgtctgtaggggtttggcgcatctgaggcatctgtcagattggccaacaccagcagaagcaggagactctggttggccagaggggaagaaagctctggagaggcagccgctttgctgcccacaccacctagtgtgaagacagtccagagtcctgctaatgacctgcagactgaaatggttgcttcctccaagagtttcaactcactactgctagttggtgcagggaaagaaaatgagagaagctgattccagaacgggtcattctcagagatagattccgtgcctgataactttttcaagtactcatttttaggaagatcgccgattctgctgctattcgatcccatcttctagcttaagcagataatttgtccttaaacctgcatttccaaaagacaacctgtctcagccggctgggggatctgctccagctccacggacccgcggacggatgggagggtggcagaggggtcaggagaagtcgctgtcgccgccgcagcccaggtggcgcacaccggctcaggcctccatgtttccacgtctcagcgggtacagatccggctccggtccggcctgcagctcggccccggctcggctccagcccgggccgcgtcggtgcggaggccaggaggcggcgagagaagaggg

SEQ ID NO: 9112 - RNA, 5642 nt, Homo sapiens
  source 1..5642: mol_type = other RNA
actggacttggagtcagaaggcctaataatcagtccctaaaatcaagtggcaactactgatattgcaggatagtgcctaggaaagaattaagagacccaaagggttgaccttgcagagactccagcctatgaagtatcagcaagtgccaaaaatttatggctctgcaaaaaagcacagggtgactcaattatgcagagagctctaccacccaatgcaaaaccctggctcccggaatctaaaggacgaaatgttgcttaaagtatgatatattaacaattccagtgcttaaaagtttccctcactaaatatttctcttggatgtaccttagcaagctcttaggaagttgctgagtgttctgatgctggtcctgtgtcctttccactttctatcgtctacttcccagctcctgtgctttccttccagagagaactgtgtgtgcagtgtactttctatgcttcaccttcagggaccttctcttctttcctttctctgtctttgtccttgagctgtgttgtctgcactgctgaatggtggcagtcctgctgcaaggttgttgttcatagattgtatgacaccagcctcaacgggtgactgtgggaactagagttagaaatctgaagctcttctgcaaagtgccttgaactcttgatagggaagatgctattgaaagggacaaattcttttaaaagtaaatattgtggcagaagtctttgttgataaaatgacacaatgcagtaacagcttcagatctggggtaaaatcagatgccaatttccatctgaacacacgatgatcctgtgttgcatcattacacatttttacttcgtgtaaaaatttctaagcaaactaatactcaaaattaatgcaagtataatgaaagtttatcattcagatttattgccatataataaatctttcacaaaaatcaggaagaagcctctggtgactttgcagagctgaggcagtgatgcacgtggtggggcctccctcctgagcgggaaccaggactgggagcatcacttgcaggcctccatggaggctgctgccccagctgagctgttagctagtgagtgcttctactgtgtgatgaatgagaaaagggaaagaggggagggcaatcagggttctgggggcacctcagtgagcccagaggcctggaggagaggctgtatgattccccagtcaggccttccttgggagtgtgccctctgtcaagatgactgggtttttgaagggcctcatttcctcacacaacaagcactgacagtcctgcagcccagggactgtcctgtggcactgcccagccctcagactcagaggacagttctgtggtcctgccagaagctcagctgttccacatgacccttaaacatttaaacaattttttggtttaaaggaaaaggaagccaatcaaaatgctttggaaacaaattaaagttgcaaattatttccccacatagtaaatacatatccttgctacctgaaatgataatcatcactccccctgctggctgagagcgcttctcctccttcagactggctctgccacaaagctaagtattagtagaagttgttgccaagcctcacctctagcctgtacatgggctctgaggtgaacacaggagtcagagtccccactccagcagtgactggaggaggcctgacagaacaagccccttggggacaggaggcaagctgcactcacctctgggaccccacccgggatgggcgctccacgagtcccttggccttagggaacctctgtttcattccatccagacgaggatagggaagcttcctgccctacctcgacagcctctaagagcacagcttggccaggccttcccgtgtggagcccacacagtggtgcactgagaggctgccagtgttttgaccttttacagagcttggggtgactgagaatggttcctccgaggccctcggaagatttgatggactcaaataacacgggcctgcagccctgggacacaggacaggagaagccagccctgacacagatgagctggcagtggattcgaacagtgtgctcagtctcgtctgggcttttgtgctttctatgttgaagaccaaatactttttctttgagaatgaaactaggctccttatctagactgtgaaggggcccgtgaggacacagagtgtgactggaaaggaaggtcccaactggccctcaatgtggccccagtggctgtttccctgcaagaagctccttcctccagctcaggcaccaacacacggatcacaccggcccagaaacaaagagcaaaacatgcttttcatcccacgtggaatacagtatgaacaaattactctcctttttctattagtgtgggtgaaggaaaaagactgttttcaaatgaagcttttctttttcccaatgattaatacagagtagattaacttaatttgtgctagactccaatttaattccagcaacagttcacaggccatattcacagaaaagttaatctgggcttcatgagaagtagccattttctttttcttttctttctttttttttttttgcgagacagggtctcactttgtggctcaggctggagtgtactggcacgttcttagctcactgcagccttgaactcctgggctcaggcaatcctcctaccttagcctcctgagtagctaggactacaggaatgtgccatcatgcctggctaatttttaagttttttgtagagatgggatctcactatgttgcccaagctggtttcagattcctgtgctcaagggattctgctaacttggctccccaaagtgctgggattacaaatgtgagccactgtatctggcccatattcttttttaagaaaagatgcagaggtgttaaatattaatatcaaattgtccaggcatggtgtttatgaaattgtgtgccctctgacaggcaaccaaacacacacgacttcatttctttattaattcctgcctcatcatcttttctcattgatgctccttaatgtcaaaggaatctctctctctcacacacacataagaccaaaacaaatatcttgaacatgcaaaaaaatagtctacgcttttgaatagtgtgcactgttgaatagtgtgcactgttggatagtgtgcactgttgaagtgtgatgtgcctaaggcaacaggatcttgggaaagctctagatttttggcttcgaaataaaactgcatgttgaatagcaggtttttacatttattattgttgtgtatttcctcccctttttgcaatactatctacgctgagttatctattgccaactagcaccaattctccaaatcaaagtgtgtgaggaaaacacactcgtgcaatcctctttaacagaagatacaccaagtaacctgtctgtctacttctgttacccagaaataaaagaacttgaagggctgcttggctggaggggtccgggtgggagagcatcctgccctcagtcggaatccatggtgaacagctggatgtcctgtggattccagtacaggccgactgctgagttgtagacaagagaccagacataggggataaaaaactcctcgggctgctcctcttccacatatttgaatttcaattctggaaatttcttcagtctgtctttgggcagcgcaacgacgccttgcttaatgatttccaggacccgttccactgacagctcagctccagcttgcagcaaccttgagctaaagaaggagatcaccagatcaatattttgcattatatcctgaaatgaaggatgagttcgaaattgttcaaagagatcgcgtttgtaaagcagggcgtataccaagtttgggttgtggtgaagggaatttgtcaggcaggagttgatgatctctaacatcattcgaatcacttcttcaatgacatttaggtcttgtgcataatctggtagaggaacatcattagaactcagcgaacctctcaaggactgtgtggcttgttccagaactttgttgtgttttttagacagcaaagaaaataaactgatgatcctctgggcagcatactgatggagagaacgaaactgtgccgacatatttgctaaagctgccaaacaatttgtgtgaaggtacttgtctcgtgtcctagtcatgttgtattgaatggttcttattaccaccaggatcaggagactccccaaggagatttcagttaaaactcgttctgaataccaagtaatattttttagtatcacttcatgaatggatctgttgaagccatcatcttccgtaaggatcaacaatattataagggccatatacacatggtgtgaattcctttcttcaacatgatacagaatctcaagaattggtaaaacaagattttccatatctgtgcgagccaacatgtatgttctaatattactattttgatggagcaaggtatacaagaggagagttgcttgatcagatgtctgctgttcacaaagagctgtgtacaaactattaaagttgatctggaaggcatgtggaattgatgaggggaaaggactgctatcttgtgtgttcttgaaggacataatggcttgtctgtaggggtttggcgcatctgaggcatctgtcagattggccaacaccagcagaagcaggagactctggttggccagaggggaagaaagctctggagaggcagccgctttgctgcccacaccacctagtgtgaagacagtccagagtcctgttgctactcctgatgcaagtccataaagcagtcctcccccatccgactgctgagggaaaacatgggcccctggaggaggtggcttttcttgtctgataaagttatataataaggtcttcacaagtttgctggtgtatggaagaaagagtggaatatcagtgatcaactgcatcaaacagcacagcaattcttccaaaagatcttctgagtcagaactgtaattgccaggagatttttcttcataagtaaaatgaagttgtaattcctcctctgacatctgacagatgaacactttcagcaaacagcaaataataaacaaagcattgtgtgtctgccaaatgaagatgtggttctgacattctgctgaaagttttagttctttggttctagaaaggaagaccttaattagtgcaccaagatttcctgttcgaggattgttttcaactaatgacctgcagactgaaatggttgcttcctccaagagtttcaactcactactgctagttggtgcagggaaagaaaatgagagaagctgattccagaacgggtcattctcagagatagattccgtgcctgataactttttcaagtactcatttttaggaagatcgccgattctgctgctattcgatcccatcttctagcttaagcagataatttgtccttaaacctgcatttccaaaagacaacctgtctcagccggctgggggatctgctccagctccacggacccgcggacggatgggagggtggcagaggggtcaggagaagtcgctgtcgccgccgcagcccaggtggcgcacaccggctcaggcctccatgtttccacgtctcagcgggtacagatccggctccggtccggcctgcagctcggccccggctcggctccagcccgggccgcgtcggtgcggaggccaggaggcggcgagagaagaggg

SEQ ID NO: 9113 - RNA, 5540 nt, Homo sapiens
  source 1..5540: mol_type = other RNA
actggacttggagtcagaaggcctaataatcagtccctaaaatcaagtggcaactactgatattgcaggatagtgcctaggaaagaattaagagacccaaagggttgaccttgcagagactccagcctatgaagtatcagcaagtgccaaaaatttatggctctgcaaaaaagcacagggtgactcaattatgcagagagctctaccacccaatgcaaaaccctggctcccggaatctaaaggacgaaatgttgcttaaagtatgatatattaacaattccagtgcttaaaagtttccctcactaaatatttctcttggatgtaccttagcaagctcttaggaagttgctgagtgttctgatgctggtcctgtgtcctttccactttctatcgtctacttcccagctcctgtgctttccttccagagagaactgtgtgtgcagtgtactttctatgcttcaccttcagggaccttctcttctttcctttctctgtctttgtccttgagctgtgttgtctgcactgctgaatggtggcagtcctgctgcaaggttgttgttcatagattgtatgacaccagcctcaacgggtgactgtgggaactagagttagaaatctgaagctcttctgcaaagtgccttgaactcttgatagggaagatgctattgaaagggacaaattcttttaaaagtaaatattgtggcagaagtctttgttgataaaatgacacaatgcagtaacagcttcagatctggggtaaaatcagatgccaatttccatctgaacacacgatgatcctgtgttgcatcattacacatttttacttcgtgtaaaaatttctaagcaaactaatactcaaaattaatgcaagtataatgaaagtttatcattcagatttattgccatataataaatctttcacaaaaatcaggaagaagcctctggtgactttgcagagctgaggcagtgatgcacgtggtggggcctccctcctgagcgggaaccaggactgggagcatcacttgcaggcctccatggaggctgctgccccagctgagctgttagctagtgagtgcttctactgtgtgatgaatgagaaaagggaaagaggggagggcaatcagggttctgggggcacctcagtgagcccagaggcctggaggagaggctgtatgattccccagtcaggccttccttgggagtgtgccctctgtcaagatgactgggtttttgaagggcctcatttcctcacacaacaagcactgacagtcctgcagcccagggactgtcctgtggcactgcccagccctcagactcagaggacagttctgtggtcctgccagaagctcagctgttccacatgacccttaaacatttaaacaattttttggtttaaaggaaaaggaagccaatcaaaatgctttggaaacaaattaaagttgcaaattatttccccacatagtaaatacatatccttgctacctgaaatgataatcatcactccccctgctggctgagagcgcttctcctccttcagactggctctgccacaaagctaagtattagtagaagttgttgccaagcctcacctctagcctgtacatgggctctgaggtgaacacaggagtcagagtccccactccagcagtgactggaggaggcctgacagaacaagccccttggggacaggaggcaagctgcactcacctctgggaccccacccgggatgggcgctccacgagtcccttggccttagggaacctctgtttcattccatccagacgaggatagggaagcttcctgccctacctcgacagcctctaagagcacagcttggccaggccttcccgtgtggagcccacacagtggtgcactgagaggctgccagtgttttgaccttttacagagcttggggtgactgagaatggttcctccgaggccctcggaagatttgatggactcaaataacacgggcctgcagccctgggacacaggacaggagaagccagccctgacacagatgagctggcagtggattcgaacagtgtgctcagtctcgtctgggcttttgtgctttctatgttgaagaccaaatactttttctttgagaatgaaactaggctccttatctagactgtgaaggggcccgtgaggacacagagtgtgactggaaaggaaggtcccaactggccctcaatgtggccccagtggctgtttccctgcaagaagctccttcctccagctcaggcaccaacacacggatcacaccggcccagaaacaaagagcaaaacatgcttttcatcccacgtggaatacagtatgaacaaattactctcctttttctattagtgtgggtgaaggaaaaagactgttttcaaatgaagcttttctttttcccaatgattaatacagagtagattaacttaatttgtgctagactccaatttaattccagcaacagttcacaggccatattcacagaaaagttaatctgggcttcatgagaagtagccattttctttttcttttctttctttttttttttttgcgagacagggtctcactttgtggctcaggctggagtgtactggcacgttcttagctcactgcagccttgaactcctgggctcaggcaatcctcctaccttagcctcctgagtagctaggactacaggaatgtgccatcatgcctggctaatttttaagttttttgtagagatgggatctcactatgttgcccaagctggtttcagattcctgtgctcaagggattctgctaacttggctccccaaagtgctgggattacaaatgtgagccactgtatctggcccatattcttttttaagaaaagatgcagaggtgttaaatattaatatcaaattgtccaggcatggtgtttatgaaattgtgtgccctctgacaggcaaccaaacacacacgacttcatttctttattaattcctgcctcatcatcttttctcattgatgctccttaatgtcaaaggaatctctctctctcacacacacataagaccaaaacaaatatcttgaacatgcaaaaaaatagtctacgcttttgaatagtgtgcactgttgaatagtgtgcactgttggatagtgtgcactgttgaagtgtgatgtgcctaaggcaacaggatcttgggaaagctctagatttttggcttcgaaataaaactgcatgttgaatagcaggtttttacatttattattgttgtgtatttcctcccctttttgcaatactatctacgctgagttatctattgccaactagcaccaattctccaaatcaaagtgtgtgaggaaaacacactcgtgcaatcctctttaacagaagatacaccaagtaacctgtctgtctacttctgttacccagaaataaaagaacttgaagggctgcttggctggaggggtccgggtgggagagcatcctgccctcagtcggaatccatggtgaacagctggatgtcctgtggattccagtacaggccgactgctgagttgtagacaagagaccagacataggggataaaaaactcctcgggctgctcctcttccacatatttgaatttcaattctggaaatttcttcagtctgtctttgggcagcgcaacgacgccttgcttaatgatttccaggacccgttccactgacagctcagctccagcttgcagcaaccttgagctaaagaaggagatcaccagatcaatattttgcattatatcctgaaatgaaggatgagttcgaaattgttcaaagagatcgcgtttgtaaagcagggcgtataccaagtttgggttgtggtgaagggaatttgtcaggcaggagttgatgatctctaacatcattcgaatcacttcttcaatgacatttaggtcttgtgcataatctggtagaggaacatcattagaactcagcgaacctctcaaggactgtgtggcttgttccagaactttgttgtgttttttagacagcaaagaaaataaactgatgatcctctgggcagcatactgatggagagaacgaaactgtgccgacatatttgctaaagctgccaaacaatttgtgtgaaggtacttgtctcgtgtcctagtcatgttgtattgaatggttcttattaccaccaggatcaggagactccccaaggagatttcagttaaaactcgttctgaataccaagtaatattttttagtatcacttcatgaatggatctgttgaagccatcatcttccgtaaggatcaacaatattataagggccatatacacatggtgtgaattcctttcttcaacatgatacagaatctcaagaattggtaaaacaagattttccatatctgtgcgagccaacatgtatgttctaatattactattttgatggagcaaggtatacaagaggagagttgcttgatcagatgtctgctgttcacaaagagctgtgtacaaactattaaagttgatctggaaggcatgtggaattgatgaggggaaaggactgctatcttgtgtgttcttgaaggacataatggcttgtctgtaggggtttggcgcatctgaggcatctgtcagattggccaacaccagcagaagcaggagactctggttggccagaggggaagaaagctctggagaggcagccgctttgctgcccacaccacctagtgtgaagacagtccagagtcctgttgctactcctgatgcaagtccataaagcagtcctcccccatccgactgctgagggaaaacatgggcccctggaggaggtggcttttcttgtctgataaagttatataataaggtcttcacaagtttgctggtgtatggaagacatggacctcgcatcaaatacttgtggctgatgctctgtcgcaaaacttctttgtggaagagttggcaggaaaggaaaacaaccattgttgatatagcttctactgatatttcatatgtaatatctaagagtggaatatcagtgatcaactgcatcaaacagcacagcaattcttccaaaagatcttctgagtcagaacctaatgacctgcagactgaaatggttgcttcctccaagagtttcaactcactactgctagttggtgcagggaaagaaaatgagagaagctgattccagaacgggtcattctcagagatagattccgtgcctgataactttttcaagtactcatttttaggaagatcgccgattctgctgctattcgatcccatcttctagcttaagcagataatttgtccttaaacctgcatttccaaaagacaacctgtctcagccggctgggggatctgctccagctccacggacccgcggacggatgggagggtggcagaggggtcaggagaagtcgctgtcgccgccgcagcccaggtggcgcacaccggctcaggcctccatgtttccacgtctcagcgggtacagatccggctccggtccggcctgcagctcggccccggctcggctccagcccgggccgcgtcggtgcggaggccaggaggcggcgagagaagaggg

SEQ ID NO: 9114 - RNA, 5768 nt, Homo sapiens
  source 1..5768: mol_type = other RNA
actggacttggagtcagaaggcctaataatcagtccctaaaatcaagtggcaactactgatattgcaggatagtgcctaggaaagaattaagagacccaaagggttgaccttgcagagactccagcctatgaagtatcagcaagtgccaaaaatttatggctctgcaaaaaagcacagggtgactcaattatgcagagagctctaccacccaatgcaaaaccctggctcccggaatctaaaggacgaaatgttgcttaaagtatgatatattaacaattccagtgcttaaaagtttccctcactaaatatttctcttggatgtaccttagcaagctcttaggaagttgctgagtgttctgatgctggtcctgtgtcctttccactttctatcgtctacttcccagctcctgtgctttccttccagagagaactgtgtgtgcagtgtactttctatgcttcaccttcagggaccttctcttctttcctttctctgtctttgtccttgagctgtgttgtctgcactgctgaatggtggcagtcctgctgcaaggttgttgttcatagattgtatgacaccagcctcaacgggtgactgtgggaactagagttagaaatctgaagctcttctgcaaagtgccttgaactcttgatagggaagatgctattgaaagggacaaattcttttaaaagtaaatattgtggcagaagtctttgttgataaaatgacacaatgcagtaacagcttcagatctggggtaaaatcagatgccaatttccatctgaacacacgatgatcctgtgttgcatcattacacatttttacttcgtgtaaaaatttctaagcaaactaatactcaaaattaatgcaagtataatgaaagtttatcattcagatttattgccatataataaatctttcacaaaaatcaggaagaagcctctggtgactttgcagagctgaggcagtgatgcacgtggtggggcctccctcctgagcgggaaccaggactgggagcatcacttgcaggcctccatggaggctgctgccccagctgagctgttagctagtgagtgcttctactgtgtgatgaatgagaaaagggaaagaggggagggcaatcagggttctgggggcacctcagtgagcccagaggcctggaggagaggctgtatgattccccagtcaggccttccttgggagtgtgccctctgtcaagatgactgggtttttgaagggcctcatttcctcacacaacaagcactgacagtcctgcagcccagggactgtcctgtggcactgcccagccctcagactcagaggacagttctgtggtcctgccagaagctcagctgttccacatgacccttaaacatttaaacaattttttggtttaaaggaaaaggaagccaatcaaaatgctttggaaacaaattaaagttgcaaattatttccccacatagtaaatacatatccttgctacctgaaatgataatcatcactccccctgctggctgagagcgcttctcctccttcagactggctctgccacaaagctaagtattagtagaagttgttgccaagcctcacctctagcctgtacatgggctctgaggtgaacacaggagtcagagtccccactccagcagtgactggaggaggcctgacagaacaagccccttggggacaggaggcaagctgcactcacctctgggaccccacccgggatgggcgctccacgagtcccttggccttagggaacctctgtttcattccatccagacgaggatagggaagcttcctgccctacctcgacagcctctaagagcacagcttggccaggccttcccgtgtggagcccacacagtggtgcactgagaggctgccagtgttttgaccttttacagagcttggggtgactgagaatggttcctccgaggccctcggaagatttgatggactcaaataacacgggcctgcagccctgggacacaggacaggagaagccagccctgacacagatgagctggcagtggattcgaacagtgtgctcagtctcgtctgggcttttgtgctttctatgttgaagaccaaatactttttctttgagaatgaaactaggctccttatctagactgtgaaggggcccgtgaggacacagagtgtgactggaaaggaaggtcccaactggccctcaatgtggccccagtggctgtttccctgcaagaagctccttcctccagctcaggcaccaacacacggatcacaccggcccagaaacaaagagcaaaacatgcttttcatcccacgtggaatacagtatgaacaaattactctcctttttctattagtgtgggtgaaggaaaaagactgttttcaaatgaagcttttctttttcccaatgattaatacagagtagattaacttaatttgtgctagactccaatttaattccagcaacagttcacaggccatattcacagaaaagttaatctgggcttcatgagaagtagccattttctttttcttttctttctttttttttttttgcgagacagggtctcactttgtggctcaggctggagtgtactggcacgttcttagctcactgcagccttgaactcctgggctcaggcaatcctcctaccttagcctcctgagtagctaggactacaggaatgtgccatcatgcctggctaatttttaagttttttgtagagatgggatctcactatgttgcccaagctggtttcagattcctgtgctcaagggattctgctaacttggctccccaaagtgctgggattacaaatgtgagccactgtatctggcccatattcttttttaagaaaagatgcagaggtgttaaatattaatatcaaattgtccaggcatggtgtttatgaaattgtgtgccctctgacaggcaaccaaacacacacgacttcatttctttattaattcctgcctcatcatcttttctcattgatgctccttaatgtcaaaggaatctctctctctcacacacacataagaccaaaacaaatatcttgaacatgcaaaaaaatagtctacgcttttgaatagtgtgcactgttgaatagtgtgcactgttggatagtgtgcactgttgaagtgtgatgtgcctaaggcaacaggatcttgggaaagctctagatttttggcttcgaaataaaactgcatgttgaatagcaggtttttacatttattattgttgtgtatttcctcccctttttgcaatactatctacgctgagttatctattgccaactagcaccaattctccaaatcaaagtgtgtgaggaaaacacactcgtgcaatcctctttaacagaagatacaccaagtaacctgtctgtctacttctgttacccagaaataaaagaacttgaagggctgcttggctggaggggtccgggtgggagagcatcctgccctcagtcggaatccatggtgaacagctggatgtcctgtggattccagtacaggccgactgctgagttgtagacaagagaccagacataggggataaaaaactcctcgggctgctcctcttccacatatttgaatttcaattctggaaatttcttcagtctgtctttgggcagcgcaacgacgccttgcttaatgatttccaggacccgttccactgacagctcagctccagcttgcagcaaccttgagctaaagaaggagatcaccagatcaatattttgcattatatcctgaaatgaaggatgagttcgaaattgttcaaagagatcgcgtttgtaaagcagggcgtataccaagtttgggttgtggtgaagggaatttgtcaggcaggagttgatgatctctaacatcattcgaatcacttcttcaatgacatttaggtcttgtgcataatctggtagaggaacatcattagaactcagcgaacctctcaaggactgtgtggcttgttccagaactttgttgtgttttttagacagcaaagaaaataaactgatgatcctctgggcagcatactgatggagagaacgaaactgtgccgacatatttgctaaagctgccaaacaatttgtgtgaaggtacttgtctcgtgtcctagtcatgttgtattgaatggttcttattaccaccaggatcaggagactccccaaggagatttcagttaaaactcgttctgaataccaagtaatattttttagtatcacttcatgaatggatctgttgaagccatcatcttccgtaaggatcaacaatattataagggccatatacacatggtgtgaattcctttcttcaacatgatacagaatctcaagaattggtaaaacaagattttccatatctgtgcgagccaacatgtatgttctaatattactattttgatggagcaaggtatacaagaggagagttgcttgatcagatgtctgctgttcacaaagagctgtgtacaaactattaaagttgatctggaaggcatgtggaattgatgaggggaaaggactgctatcttgtgtgttcttgaaggacataatggcttgtctgtaggggtttggcgcatctgaggcatctgtcagattggccaacaccagcagaagcaggagactctggttggccagaggggaagaaagctctggagaggcagccgctttgctgcccacaccacctagtgtgaagacagtccagagtcctgttgctactcctgatgcaagtccataaagcagtcctcccccatccgactgctgagggaaaacatgggcccctggaggaggtggcttttcttgtctgataaagttatataataaggtcttcacaagtttgctggtgtatggaagacatggacctcgcatcaaatacttgtggctgatgctctgtcgcaaaacttctttgtggaagagttggcaggaaaggaaaacaaccattgttgatatagcttctactgatatttcatatgtaatatctaagagtggaatatcagtgatcaactgcatcaaacagcacagcaattcttccaaaagatcttctgagtcagaactgtaattgccaggagatttttcttcataagtaaaatgaagttgtaattcctcctctgacatctgacagatgaacactttcagcaaacagcaaataataaacaaagcattgtgtgtctgccaaatgaagatgtggttctgacattctgctgaaagttttagttctttggttctagaaaggaagaccttaattagtgcaccaagatttcctgttcgaggattgttttcaactaatgacctgcagactgaaatggttgcttcctccaagagtttcaactcactactgctagttggtgcagggaaagaaaatgagagaagctgattccagaacgggtcattctcagagatagattccgtgcctgataactttttcaagtactcatttttaggaagatcgccgattctgctgctattcgatcccatcttctagcttaagcagataatttgtccttaaacctgcatttccaaaagacaacctgtctcagccggctgggggatctgctccagctccacggacccgcggacggatgggagggtggcagaggggtcaggagaagtcgctgtcgccgccgcagcccaggtggcgcacaccggctcaggcctccatgtttccacgtctcagcgggtacagatccggctccggtccggcctgcagctcggccccggctcggctccagcccgggccgcgtcggtgcggaggccaggaggcggcgagagaagaggg

SEQ ID NO: 9115 - RNA, 5765 nt, Homo sapiens
  source 1..5765: mol_type = other RNA
actggacttggagtcagaaggcctaataatcagtccctaaaatcaagtggcaactactgatattgcaggatagtgcctaggaaagaattaagagacccaaagggttgaccttgcagagactccagcctatgaagtatcagcaagtgccaaaaatttatggctctgcaaaaaagcacagggtgactcaattatgcagagagctctaccacccaatgcaaaaccctggctcccggaatctaaaggacgaaatgttgcttaaagtatgatatattaacaattccagtgcttaaaagtttccctcactaaatatttctcttggatgtaccttagcaagctcttaggaagttgctgagtgttctgatgctggtcctgtgtcctttccactttctatcgtctacttcccagctcctgtgctttccttccagagagaactgtgtgtgcagtgtactttctatgcttcaccttcagggaccttctcttctttcctttctctgtctttgtccttgagctgtgttgtctgcactgctgaatggtggcagtcctgctgcaaggttgttgttcatagattgtatgacaccagcctcaacgggtgactgtgggaactagagttagaaatctgaagctcttctgcaaagtgccttgaactcttgatagggaagatgctattgaaagggacaaattcttttaaaagtaaatattgtggcagaagtctttgttgataaaatgacacaatgcagtaacagcttcagatctggggtaaaatcagatgccaatttccatctgaacacacgatgatcctgtgttgcatcattacacatttttacttcgtgtaaaaatttctaagcaaactaatactcaaaattaatgcaagtataatgaaagtttatcattcagatttattgccatataataaatctttcacaaaaatcaggaagaagcctctggtgactttgcagagctgaggcagtgatgcacgtggtggggcctccctcctgagcgggaaccaggactgggagcatcacttgcaggcctccatggaggctgctgccccagctgagctgttagctagtgagtgcttctactgtgtgatgaatgagaaaagggaaagaggggagggcaatcagggttctgggggcacctcagtgagcccagaggcctggaggagaggctgtatgattccccagtcaggccttccttgggagtgtgccctctgtcaagatgactgggtttttgaagggcctcatttcctcacacaacaagcactgacagtcctgcagcccagggactgtcctgtggcactgcccagccctcagactcagaggacagttctgtggtcctgccagaagctcagctgttccacatgacccttaaacatttaaacaattttttggtttaaaggaaaaggaagccaatcaaaatgctttggaaacaaattaaagttgcaaattatttccccacatagtaaatacatatccttgctacctgaaatgataatcatcactccccctgctggctgagagcgcttctcctccttcagactggctctgccacaaagctaagtattagtagaagttgttgccaagcctcacctctagcctgtacatgggctctgaggtgaacacaggagtcagagtccccactccagcagtgactggaggaggcctgacagaacaagccccttggggacaggaggcaagctgcactcacctctgggaccccacccgggatgggcgctccacgagtcccttggccttagggaacctctgtttcattccatccagacgaggatagggaagcttcctgccctacctcgacagcctctaagagcacagcttggccaggccttcccgtgtggagcccacacagtggtgcactgagaggctgccagtgttttgaccttttacagagcttggggtgactgagaatggttcctccgaggccctcggaagatttgatggactcaaataacacgggcctgcagccctgggacacaggacaggagaagccagccctgacacagatgagctggcagtggattcgaacagtgtgctcagtctcgtctgggcttttgtgctttctatgttgaagaccaaatactttttctttgagaatgaaactaggctccttatctagactgtgaaggggcccgtgaggacacagagtgtgactggaaaggaaggtcccaactggccctcaatgtggccccagtggctgtttccctgcaagaagctccttcctccagctcaggcaccaacacacggatcacaccggcccagaaacaaagagcaaaacatgcttttcatcccacgtggaatacagtatgaacaaattactctcctttttctattagtgtgggtgaaggaaaaagactgttttcaaatgaagcttttctttttcccaatgattaatacagagtagattaacttaatttgtgctagactccaatttaattccagcaacagttcacaggccatattcacagaaaagttaatctgggcttcatgagaagtagccattttctttttcttttctttctttttttttttttgcgagacagggtctcactttgtggctcaggctggagtgtactggcacgttcttagctcactgcagccttgaactcctgggctcaggcaatcctcctaccttagcctcctgagtagctaggactacaggaatgtgccatcatgcctggctaatttttaagttttttgtagagatgggatctcactatgttgcccaagctggtttcagattcctgtgctcaagggattctgctaacttggctccccaaagtgctgggattacaaatgtgagccactgtatctggcccatattcttttttaagaaaagatgcagaggtgttaaatattaatatcaaattgtccaggcatggtgtttatgaaattgtgtgccctctgacaggcaaccaaacacacacgacttcatttctttattaattcctgcctcatcatcttttctcattgatgctccttaatgtcaaaggaatctctctctctcacacacacataagaccaaaacaaatatcttgaacatgcaaaaaaatagtctacgcttttgaatagtgtgcactgttgaatagtgtgcactgttggatagtgtgcactgttgaagtgtgatgtgcctaaggcaacaggatcttgggaaagctctagatttttggcttcgaaataaaactgcatgttgaatagcaggtttttacatttattattgttgtgtatttcctcccctttttgcaatactatctacgctgagttatctattgccaactagcaccaattctccaaatcaaagtgtgtgaggaaaacacactcgtgcaatcctctttaacagaagatacaccaagtaacctgtctgtctacttctgttacccagaaataaaagaacttgaagggctgcttggctggaggggtccgggtgggagagcatcctgccctcagtcggaatccatggtgaacagctggatgtcctgtggattccagtacaggccgactgctgagttgtagacaagagaccagacataggggataaaaaactcctcgggctgctcctcttccacatatttgaatttcaattctggaaatttcttcagtctgtctttgggcagcgcaacgacgccttgcttaatgatttccaggacccgttccactgacagctcagctccagcttgcagcaaccttgagctaaagaaggagatcaccagatcaatattttgcattatatcctgaaatgaaggatgagttcgaaattgttcaaagagatcgcgtttgtaaagcagggcgtataccaagtttgggttgtggtgaagggaatttgtcaggcaggagttgatgatctctaacatcattcgaatcacttcttcaatgacatttaggtcttgtgcataatctggtagaggaacatcattagaactcagcgaacctctcaaggactgtgtggcttgttccagaactttgttgtgttttttagacagcaaagaaaataaactgatgatcctctgggcagcatactgatggagagaacgaaactgtgccgacatatttgctaaagctgccaaacaatttgtgtgaaggtacttgtctcgtgtcctagtcatgttgtattgaatggttcttattaccaccaggatcaggagactccccaaggagatttcagttaaaactcgttctgaataccaagtaatattttttagtatcacttcatgaatggatctgttgaagccatcatcttccgtaaggatcaacaatattataagggccatatacacatggtgtgaattcctttcttcaacatgatacagaatctcaagaattggtaaaacaagattttccatatctgtgcgagccaacatgtatgttctaatattactattttgatggagcaaggtatacaagaggagagttgcttgatcagatgtctgctgttcacaaagagctgtgtacaaactattaaagttgatctggaaggcatgtggaattgatgaggggaaaggactgctatcttgtgtgttcttgaaggacataatggcttgtctgtaggggtttggcgcatctgaggcatctgtcagattggccaacaccagcagaagcaggagactctggttggccagaggggaagaaagctctggagaggcagccgctttgctgcccacaccacctagtgtgaagacagtccagagtcctgttgctactcctgatgcaagtccataaagcagtcctcccccatccgactgctgagggaaaacatgggcccctggaggaggtggcttttcttgtctgataaagttatataataaggtcttcacaagtttgctggtgtatggaagacatggacctcgcatcaaatacttgtggctgatgctctgtcgcaaaacttctttgtggaagagttggcaggaaaggaaaacaaccattgttgatatagcttctactgatatttcatatgtaatatctaagagtggaatatcagtgatcaactgcatcaaacagcacagcaattcttccaaaagatcttctgagtcagaactgtaattgccaggagatttttcttcataagtaaaatgaagttgtaattcctcctctgacatctgacagatgaacactttcagcaaacagcaaataataaacaaagcattgtgtgtctgccaaatgaagatgtggttctgacattctgctgaaagttttagttctttggttctagaaaggaagaccttaattagtgcaccaagatttcctgttcgaggattgttttcaactaatgacctgcagactgaaatggttgcttcctccaagagtttcaactcactgctagttggtgcagggaaagaaaatgagagaagctgattccagaacgggtcattctcagagatagattccgtgcctgataactttttcaagtactcatttttaggaagatcgccgattctgctgctattcgatcccatcttctagcttaagcagataatttgtccttaaacctgcatttccaaaagacaacctgtctcagccggctgggggatctgctccagctccacggacccgcggacggatgggagggtggcagaggggtcaggagaagtcgctgtcgccgccgcagcccaggtggcgcacaccggctcaggcctccatgtttccacgtctcagcgggtacagatccggctccggtccggcctgcagctcggccccggctcggctccagcccgggccgcgtcggtgcggaggccaggaggcggcgagagaagaggg

SEQ ID NO: 9116 - RNA, 5765 nt, Homo sapiens
  source 1..5765: mol_type = other RNA
actggacttggagtcagaaggcctaataatcagtccctaaaatcaagtggcaactactgatattgcaggatagtgcctaggaaagaattaagagacccaaagggttgaccttgcagagactccagcctatgaagtatcagcaagtgccaaaaatttatggctctgcaaaaaagcacagggtgactcaattatgcagagagctctaccacccaatgcaaaaccctggctcccggaatctaaaggacgaaatgttgcttaaagtatgatatattaacaattccagtgcttaaaagtttccctcactaaatatttctcttggatgtaccttagcaagctcttaggaagttgctgagtgttctgatgctggtcctgtgtcctttccactttctatcgtctacttcccagctcctgtgctttccttccagagagaactgtgtgtgcagtgtactttctatgcttcaccttcagggaccttctcttctttcctttctctgtctttgtccttgagctgtgttgtctgcactgctgaatggtggcagtcctgctgcaaggttgttgttcatagattgtatgacaccagcctcaacgggtgactgtgggaactagagttagaaatctgaagctcttctgcaaagtgccttgaactcttgatagggaagatgctattgaaagggacaaattcttttaaaagtaaatattgtggcagaagtctttgttgataaaatgacacaatgcagtaacagcttcagatctggggtaaaatcagatgccaatttccatctgaacacacgatgatcctgtgttgcatcattacacatttttacttcgtgtaaaaatttctaagcaaactaatactcaaaattaatgcaagtataatgaaagtttatcattcagatttattgccatataataaatctttcacaaaaatcaggaagaagcctctggtgactttgcagagctgaggcagtgatgcacgtggtggggcctccctcctgagcgggaaccaggactgggagcatcacttgcaggcctccatggaggctgctgccccagctgagctgttagctagtgagtgcttctactgtgtgatgaatgagaaaagggaaagaggggagggcaatcagggttctgggggcacctcagtgagcccagaggcctggaggagaggctgtatgattccccagtcaggccttccttgggagtgtgccctctgtcaagatgactgggtttttgaagggcctcatttcctcacacaacaagcactgacagtcctgcagcccagggactgtcctgtggcactgcccagccctcagactcagaggacagttctgtggtcctgccagaagctcagctgttccacatgacccttaaacatttaaacaattttttggtttaaaggaaaaggaagccaatcaaaatgctttggaaacaaattaaagttgcaaattatttccccacatagtaaatacatatccttgctacctgaaatgataatcatcactccccctgctggctgagagcgcttctcctccttcagactggctctgccacaaagctaagtattagtagaagttgttgccaagcctcacctctagcctgtacatgggctctgaggtgaacacaggagtcagagtccccactccagcagtgactggaggaggcctgacagaacaagccccttggggacaggaggcaagctgcactcacctctgggaccccacccgggatgggcgctccacgagtcccttggccttagggaacctctgtttcattccatccagacgaggatagggaagcttcctgccctacctcgacagcctctaagagcacagcttggccaggccttcccgtgtggagcccacacagtggtgcactgagaggctgccagtgttttgaccttttacagagcttggggtgactgagaatggttcctccgaggccctcggaagatttgatggactcaaataacacgggcctgcagccctgggacacaggacaggagaagccagccctgacacagatgagctggcagtggattcgaacagtgtgctcagtctcgtctgggcttttgtgctttctatgttgaagaccaaatactttttctttgagaatgaaactaggctccttatctagactgtgaaggggcccgtgaggacacagagtgtgactggaaaggaaggtcccaactggccctcaatgtggccccagtggctgtttccctgcaagaagctccttcctccagctcaggcaccaacacacggatcacaccggcccagaaacaaagagcaaaacatgcttttcatcccacgtggaatacagtatgaacaaattactctcctttttctattagtgtgggtgaaggaaaaagactgttttcaaatgaagcttttctttttcccaatgattaatacagagtagattaacttaatttgtgctagactccaatttaattccagcaacagttcacaggccatattcacagaaaagttaatctgggcttcatgagaagtagccattttctttttcttttctttctttttttttttttgcgagacagggtctcactttgtggctcaggctggagtgtactggcacgttcttagctcactgcagccttgaactcctgggctcaggcaatcctcctaccttagcctcctgagtagctaggactacaggaatgtgccatcatgcctggctaatttttaagttttttgtagagatgggatctcactatgttgcccaagctggtttcagattcctgtgctcaagggattctgctaacttggctccccaaagtgctgggattacaaatgtgagccactgtatctggcccatattcttttttaagaaaagatgcagaggtgttaaatattaatatcaaattgtccaggcatggtgtttatgaaattgtgtgccctctgacaggcaaccaaacacacacgacttcatttctttattaattcctgcctcatcatcttttctcattgatgctccttaatgtcaaaggaatctctctctctcacacacacataagaccaaaacaaatatcttgaacatgcaaaaaaatagtctacgcttttgaatagtgtgcactgttgaatagtgtgcactgttggatagtgtgcactgttgaagtgtgatgtgcctaaggcaacaggatcttgggaaagctctagatttttggcttcgaaataaaactgcatgttgaatagcaggtttttacatttattattgttgtgtatttcctcccctttttgcaatactatctacgctgagttatctattgccaactagcaccaattctccaaatcaaagtgtgtgaggaaaacacactcgtgcaatcctctttaacagaagatacaccaagtaacctgtctgtctacttctgttacccagaaataaaagaacttgaagggctgcttggctggaggggtccgggtgggagagcatcctgccctcagtcggaatccatggtgaacagctggatgtcctgtggattccagtacaggccgactgctgagttgtagacaagagaccagacataggggataaaaaactcctcgggctgctcctcttccacatatttgaatttcaattctggaaatttcttcagtctgtctttgggcagcgcaacgacgccttgcttaatgatttccaggacccgttccactgacagctcagctccagcttgcagcaaccttgagctaaagaaggagatcaccagatcaatattttgcattatatcctgaaatgaaggatgagttcgaaattgttcaaagagatcgcgtttgtaaagcagggcgtataccaagtttgggttgtggtgaagggaatttgtcaggcaggagttgatgatctctaacatcattcgaatcacttcttcaatgacatttaggtcttgtgcataatctggtagaggaacatcattagaactcagcgaacctctcaaggactgtgtggcttgttccagaactttgttgtgttttttagacagcaaagaaaataaactgatgatcctctgggcagcatactgatggagagaacgaaactgtgccgacatatttgctaaagctgccaaacaatttgtgtgaaggtacttgtctcgtgtcctagtcatgttgtattgaatggttcttattaccaccaggatcaggagactccccaaggagatttcagttaaaactcgttctgaataccaagtaatattttttagtatcacttcatgaatggatctgttgaagccatcatcttccgtaaggatcaacaatattataagggccatatacacatggtgtgaattcctttcttcaacatgatacagaatctcaagaattggtaaaacaagattttccatatctgtgcgagccaacatgtatgttctaatattactattttgatggagcaaggtatacaagaggagagttgcttgatcagatgtctgctgttcacaaagagctgtgtacaaactattaaagttgatctggaaggcatgtggaattgatgaggggaaaggactgctatcttgtgtgttcttgaaggacataatggcttgtctgtaggggtttggcgcatctgaggcatctgtcagattggccaacaccagcagaagcaggagactctggttggccagaggggaagaaagctctggagaggcagccgctttgctgcccacaccacctagtgtgaagacagtccagagtcttgctactcctgatgcaagtccataaagcagtcctcccccatccgactgctgagggaaaacatgggcccctggaggaggtggcttttcttgtctgataaagttatataataaggtcttcacaagtttgctggtgtatggaagacatggacctcgcatcaaatacttgtggctgatgctctgtcgcaaaacttctttgtggaagagttggcaggaaaggaaaacaaccattgttgatatagcttctactgatatttcatatgtaatatctaagagtggaatatcagtgatcaactgcatcaaacagcacagcaattcttccaaaagatcttctgagtcagaactgtaattgccaggagatttttcttcataagtaaaatgaagttgtaattcctcctctgacatctgacagatgaacactttcagcaaacagcaaataataaacaaagcattgtgtgtctgccaaatgaagatgtggttctgacattctgctgaaagttttagttctttggttctagaaaggaagaccttaattagtgcaccaagatttcctgttcgaggattgttttcaactaatgacctgcagactgaaatggttgcttcctccaagagtttcaactcactactgctagttggtgcagggaaagaaaatgagagaagctgattccagaacgggtcattctcagagatagattccgtgcctgataactttttcaagtactcatttttaggaagatcgccgattctgctgctattcgatcccatcttctagcttaagcagataatttgtccttaaacctgcatttccaaaagacaacctgtctcagccggctgggggatctgctccagctccacggacccgcggacggatgggagggtggcagaggggtcaggagaagtcgctgtcgccgccgcagcccaggtggcgcacaccggctcaggcctccatgtttccacgtctcagcgggtacagatccggctccggtccggcctgcagctcggccccggctcggctccagcccgggccgcgtcggtgcggaggccaggaggcggcgagagaagaggg

SEQ ID NO: 9117 - RNA, 5585 nt, Homo sapiens
  source 1..5585: mol_type = other RNA
actggacttggagtcagaaggcctaataatcagtccctaaaatcaagtggcaactactgatattgcaggatagtgcctaggaaagaattaagagacccaaagggttgaccttgcagagactccagcctatgaagtatcagcaagtgccaaaaatttatggctctgcaaaaaagcacagggtgactcaattatgcagagagctctaccacccaatgcaaaaccctggctcccggaatctaaaggacgaaatgttgcttaaagtatgatatattaacaattccagtgcttaaaagtttccctcactaaatatttctcttggatgtaccttagcaagctcttaggaagttgctgagtgttctgatgctggtcctgtgtcctttccactttctatcgtctacttcccagctcctgtgctttccttccagagagaactgtgtgtgcagtgtactttctatgcttcaccttcagggaccttctcttctttcctttctctgtctttgtccttgagctgtgttgtctgcactgctgaatggtggcagtcctgctgcaaggttgttgttcatagattgtatgacaccagcctcaacgggtgactgtgggaactagagttagaaatctgaagctcttctgcaaagtgccttgaactcttgatagggaagatgctattgaaagggacaaattcttttaaaagtaaatattgtggcagaagtctttgttgataaaatgacacaatgcagtaacagcttcagatctggggtaaaatcagatgccaatttccatctgaacacacgatgatcctgtgttgcatcattacacatttttacttcgtgtaaaaatttctaagcaaactaatactcaaaattaatgcaagtataatgaaagtttatcattcagatttattgccatataataaatctttcacaaaaatcaggaagaagcctctggtgactttgcagagctgaggcagtgatgcacgtggtggggcctccctcctgagcgggaaccaggactgggagcatcacttgcaggcctccatggaggctgctgccccagctgagctgttagctagtgagtgcttctactgtgtgatgaatgagaaaagggaaagaggggagggcaatcagggttctgggggcacctcagtgagcccagaggcctggaggagaggctgtatgattccccagtcaggccttccttgggagtgtgccctctgtcaagatgactgggtttttgaagggcctcatttcctcacacaacaagcactgacagtcctgcagcccagggactgtcctgtggcactgcccagccctcagactcagaggacagttctgtggtcctgccagaagctcagctgttccacatgacccttaaacatttaaacaattttttggtttaaaggaaaaggaagccaatcaaaatgctttggaaacaaattaaagttgcaaattatttccccacatagtaaatacatatccttgctacctgaaatgataatcatcactccccctgctggctgagagcgcttctcctccttcagactggctctgccacaaagctaagtattagtagaagttgttgccaagcctcacctctagcctgtacatgggctctgaggtgaacacaggagtcagagtccccactccagcagtgactggaggaggcctgacagaacaagccccttggggacaggaggcaagctgcactcacctctgggaccccacccgggatgggcgctccacgagtcccttggccttagggaacctctgtttcattccatccagacgaggatagggaagcttcctgccctacctcgacagcctctaagagcacagcttggccaggccttcccgtgtggagcccacacagtggtgcactgagaggctgccagtgttttgaccttttacagagcttggggtgactgagaatggttcctccgaggccctcggaagatttgatggactcaaataacacgggcctgcagccctgggacacaggacaggagaagccagccctgacacagatgagctggcagtggattcgaacagtgtgctcagtctcgtctgggcttttgtgctttctatgttgaagaccaaatactttttctttgagaatgaaactaggctccttatctagactgtgaaggggcccgtgaggacacagagtgtgactggaaaggaaggtcccaactggccctcaatgtggccccagtggctgtttccctgcaagaagctccttcctccagctcaggcaccaacacacggatcacaccggcccagaaacaaagagcaaaacatgcttttcatcccacgtggaatacagtatgaacaaattactctcctttttctattagtgtgggtgaaggaaaaagactgttttcaaatgaagcttttctttttcccaatgattaatacagagtagattaacttaatttgtgctagactccaatttaattccagcaacagttcacaggccatattcacagaaaagttaatctgggcttcatgagaagtagccattttctttttcttttctttctttttttttttttgcgagacagggtctcactttgtggctcaggctggagtgtactggcacgttcttagctcactgcagccttgaactcctgggctcaggcaatcctcctaccttagcctcctgagtagctaggactacaggaatgtgccatcatgcctggctaatttttaagttttttgtagagatgggatctcactatgttgcccaagctggtttcagattcctgtgctcaagggattctgctaacttggctccccaaagtgctgggattacaaatgtgagccactgtatctggcccatattcttttttaagaaaagatgcagaggtgttaaatattaatatcaaattgtccaggcatggtgtttatgaaattgtgtgccctctgacaggcaaccaaacacacacgacttcatttctttattaattcctgcctcatcatcttttctcattgatgctccttaatgtcaaaggaatctctctctctcacacacacataagaccaaaacaaatatcttgaacatgcaaaaaaatagtctacgcttttgaatagtgtgcactgttgaatagtgtgcactgttggatagtgtgcactgttgaagtgtgatgtgcctaaggcaacaggatcttgggaaagctctagatttttggcttcgaaataaaactgcatgttgaatagcaggtttttacatttattattgttgtgtatttcctcccctttttgcaatactatctacgctgagttatctattgccaactagcaccaattctccaaatcaaagtgtgtgaggaaaacacactcgtgcaatcctctttaacagaagatacaccaagtaacctgtctgtctacttctgttacccagaaataaaagaacttgaagggctgcttggctggaggggtccgggtgggagagcatcctgccctcagtcggaatccatggtgaacagctggatgtcctgtggattccagtacaggccgactgctgagttgtagacaagagaccagacataggggataaaaaactcctcgggctgctcctcttccacatatttgaatttcaattctggaaatttcttcagtctgtctttgggcagcgcaacgacgccttgcttaatgatttccaggacccgttccactgacagctcagctccagcttgcagcaaccttgagctaaagaaggagatcaccagatcaatattttgcattatatcctgaaatgaaggatgagttcgaaattgttcaaagagatcgcgtttgtaaagcagggcgtataccaagtttgggttgtggtgaagggaatttgtcaggcaggagttgatgatctctaacatcattcgaatcacttcttcaatgacatttaggtcttgtgcataatctggtagaggaacatcattagaactcagcgaacctctcaaggactgtgtggcttgttccagaactttgttgtgttttttagacagcaaagaaaataaactgatgatcctctgggcagcatactgatggagagaacgaaactgtgccgacatatttgctaaagctgccaaacaatttgtgtgaaggtacttgtctcgtgtcctagtcatgttgtattgaatggttcttattaccaccaggatcaggagactccccaaggagatttcagttaaaactcgttctgaataccaagtaatattttttagtatcacttcatgaatggatctgttgaagccatcatcttccgtaaggatcaacaatattataagggccatatacacatggtgtgaattcctttcttcaacatgatacagaatctcaagaattggtaaaacaagattttccatatctgtgcgagccaacatgtatgttctaatattactattttgatggagcaaggtatacaagaggagagttgcttgatcagatgtctgctgttcacaaagagctgtgtacaaactattaaagttgatctggaaggcatgtggaattgatgaggggaaaggactgctatttgctactcctgatgcaagtccataaagcagtcctcccccatccgactgctgagggaaaacatgggcccctggaggaggtggcttttcttgtctgataaagttatataataaggtcttcacaagtttgctggtgtatggaagacatggacctcgcatcaaatacttgtggctgatgctctgtcgcaaaacttctttgtggaagagttggcaggaaaggaaaacaaccattgttgatatagcttctactgatatttcatatgtaatatctaagagtggaatatcagtgatcaactgcatcaaacagcacagcaattcttccaaaagatcttctgagtcagaactgtaattgccaggagatttttcttcataagtaaaatgaagttgtaattcctcctctgacatctgacagatgaacactttcagcaaacagcaaataataaacaaagcattgtgtgtctgccaaatgaagatgtggttctgacattctgctgaaagttttagttctttggttctagaaaggaagaccttaattagtgcaccaagatttcctgttcgaggattgttttcaactaatgacctgcagactgaaatggttgcttcctccaagagtttcaactcactactgctagttggtgcagggaaagaaaatgagagaagctgattccagaacgggtcattctcagagatagattccgtgcctgataactttttcaagtactcatttttaggaagatcgccgattctgctgctattcgatcccatcttctagcttaagcagataatttgtccttaaacctgcatttccaaaagacaacctgtctcagccggctgggggatctgctccagctccacggacccgcggacggatgggagggtggcagaggggtcaggagaagtcgctgtcgccgccgcagcccaggtggcgcacaccggctcaggcctccatgtttccacgtctcagcgggtacagatccggctccggtccggcctgcagctcggccccggctcggctccagcccgggccgcgtcggtgcggaggccaggaggcggcgagagaagaggg

SEQ ID NO: 9118 - RNA, 5363 nt, Homo sapiens
  source 1..5363: mol_type = other RNA
actggacttggagtcagaaggcctaataatcagtccctaaaatcaagtggcaactactgatattgcaggatagtgcctaggaaagaattaagagacccaaagggttgaccttgcagagactccagcctatgaagtatcagcaagtgccaaaaatttatggctctgcaaaaaagcacagggtgactcaattatgcagagagctctaccacccaatgcaaaaccctggctcccggaatctaaaggacgaaatgttgcttaaagtatgatatattaacaattccagtgcttaaaagtttccctcactaaatatttctcttggatgtaccttagcaagctcttaggaagttgctgagtgttctgatgctggtcctgtgtcctttccactttctatcgtctacttcccagctcctgtgctttccttccagagagaactgtgtgtgcagtgtactttctatgcttcaccttcagggaccttctcttctttcctttctctgtctttgtccttgagctgtgttgtctgcactgctgaatggtggcagtcctgctgcaaggttgttgttcatagattgtatgacaccagcctcaacgggtgactgtgggaactagagttagaaatctgaagctcttctgcaaagtgccttgaactcttgatagggaagatgctattgaaagggacaaattcttttaaaagtaaatattgtggcagaagtctttgttgataaaatgacacaatgcagtaacagcttcagatctggggtaaaatcagatgccaatttccatctgaacacacgatgatcctgtgttgcatcattacacatttttacttcgtgtaaaaatttctaagcaaactaatactcaaaattaatgcaagtataatgaaagtttatcattcagatttattgccatataataaatctttcacaaaaatcaggaagaagcctctggtgactttgcagagctgaggcagtgatgcacgtggtggggcctccctcctgagcgggaaccaggactgggagcatcacttgcaggcctccatggaggctgctgccccagctgagctgttagctagtgagtgcttctactgtgtgatgaatgagaaaagggaaagaggggagggcaatcagggttctgggggcacctcagtgagcccagaggcctggaggagaggctgtatgattccccagtcaggccttccttgggagtgtgccctctgtcaagatgactgggtttttgaagggcctcatttcctcacacaacaagcactgacagtcctgcagcccagggactgtcctgtggcactgcccagccctcagactcagaggacagttctgtggtcctgccagaagctcagctgttccacatgacccttaaacatttaaacaattttttggtttaaaggaaaaggaagccaatcaaaatgctttggaaacaaattaaagttgcaaattatttccccacatagtaaatacatatccttgctacctgaaatgataatcatcactccccctgctggctgagagcgcttctcctccttcagactggctctgccacaaagctaagtattagtagaagttgttgccaagcctcacctctagcctgtacatgggctctgaggtgaacacaggagtcagagtccccactccagcagtgactggaggaggcctgacagaacaagccccttggggacaggaggcaagctgcactcacctctgggaccccacccgggatgggcgctccacgagtcccttggccttagggaacctctgtttcattccatccagacgaggatagggaagcttcctgccctacctcgacagcctctaagagcacagcttggccaggccttcccgtgtggagcccacacagtggtgcactgagaggctgccagtgttttgaccttttacagagcttggggtgactgagaatggttcctccgaggccctcggaagatttgatggactcaaataacacgggcctgcagccctgggacacaggacaggagaagccagccctgacacagatgagctggcagtggattcgaacagtgtgctcagtctcgtctgggcttttgtgctttctatgttgaagaccaaatactttttctttgagaatgaaactaggctccttatctagactgtgaaggggcccgtgaggacacagagtgtgactggaaaggaaggtcccaactggccctcaatgtggccccagtggctgtttccctgcaagaagctccttcctccagctcaggcaccaacacacggatcacaccggcccagaaacaaagagcaaaacatgcttttcatcccacgtggaatacagtatgaacaaattactctcctttttctattagtgtgggtgaaggaaaaagactgttttcaaatgaagcttttctttttcccaatgattaatacagagtagattaacttaatttgtgctagactccaatttaattccagcaacagttcacaggccatattcacagaaaagttaatctgggcttcatgagaagtagccattttctttttcttttctttctttttttttttttgcgagacagggtctcactttgtggctcaggctggagtgtactggcacgttcttagctcactgcagccttgaactcctgggctcaggcaatcctcctaccttagcctcctgagtagctaggactacaggaatgtgccatcatgcctggctaatttttaagttttttgtagagatgggatctcactatgttgcccaagctggtttcagattcctgtgctcaagggattctgctaacttggctccccaaagtgctgggattacaaatgtgagccactgtatctggcccatattcttttttaagaaaagatgcagaggtgttaaatattaatatcaaattgtccaggcatggtgtttatgaaattgtgtgccctctgacaggcaaccaaacacacacgacttcatttctttattaattcctgcctcatcatcttttctcattgatgctccttaatgtcaaaggaatctctctctctcacacacacataagaccaaaacaaatatcttgaacatgcaaaaaaatagtctacgcttttgaatagtgtgcactgttgaatagtgtgcactgttggatagtgtgcactgttgaagtgtgatgtgcctaaggcaacaggatcttgggaaagctctagatttttggcttcgaaataaaactgcatgttgaatagcaggtttttacatttattattgttgtgtatttcctcccctttttgcaatactatctacgctgagttatctattgccaactagcaccaattctccaaatcaaagtgtgtgaggaaaacacactcgtgcaatcctctttaacagaagatacaccaagtaacctgtctgtctacttctgttacccagaaataaaagaacttgaagggctgcttggctggaggggtccgggtgggagagcatcctgccctcagtcggaatccatggtgaacagctggatgtcctgtggattccagtacaggccgactgctgagttgtagacaagagaccagacataggggataaaaaactcctcgggctgctcctcttccacatatttgaatttcaattctggaaatttcttcagtctgtctttgggcagcgcaacgacgccttgcttaatgatttccaggacccgttccactgacagctcagctccagcttgcagcaaccttgagctaaagaaggagatcaccagatcaatattttgcattatatcctgaaatgaaggatgagttcgaaattgttcaaagagatcgcgtttgtaaagcagggcgtataccaagtttgggttgtggtgaagggaatttgtcaggcaggagttgatgatctctaacatcattcgaatcacttcttcaatgacatttaggtcttgtgcataatctggtagaggaacatcattagaactcagcgaacctctcaaggactgtgtggcttgttccagaactttgttgtgttttttagacagcaaagaaaataaactggaagcataggatctgagaatgtgagagcaagttaaagacaagagttcctctccattgtcactgagggtcgagaagcaatgctgaagcgtagaacagtgagagtgggggaaatacagtttgtccaacacataaacatatctccgcaagtggcggcaggtataactgatgatcctctgggcagcatactgatggagagaacgaaactgtgccgacatatttgctaaagctgccaaacaatttgtgtgaaggtacttgtctcgtgtcctagtcatgttgtattgaatggttcttattaccaccaggatcaggagactccccaaggagatttcagttaaaactcgttctgaataccaagtaatattttttagtatcacttcatgaatggatctgttgaagccatcatcttccgtaaggatcaacaatattataagggccatatacacatggtgtgaattcctttcttcaacatgatacagaatctcaagaattggtaaaacaagattttccatatctgtgcgagccaacatgtatgttctaatattactattttgatggagcaaggtatacaagaggagagttgcttgatcagatgtctgctgttcacaaagagctgtgtacaaactattaaagttgatctggaaggcatgtggaattgatgaggggaaaggactgctatcttgtgtgttcttgaaggacataatggcttgtctgtaggggtttggcgcatctgaggcatctgtcagattggccaacaccagcagaagcaggagactctggttggccagaggggaagaaagctctggagaggcagccgctttgctgcccacaccacctagtgtgaagacagtccagagtcctgctaatgacctgcagactgaaatggttgcttcctccaagagtttcaactcactactgctagttggtgcagggaaagaaaatgagagaagctgattccagaacgggtcattctcagagatagattccgtgcctgataactttttcaagtactcatttttaggaagatcgccgattctgctgctattcgatcccatcttctagcttaagcagataatttgtccttaaacctgcatttccaaaagacaacctgtctcagccggctgggggatctgctccagctccacggacccgcggacggatgggagggtggcagaggggtcaggagaagtcgctgtcgccgccgcagcccaggtggcgcacaccggctcaggcctccatgtttccacgtctcagcgggtacagatccggctccggtccggcctgcagctcggccccggctcggctccagcccgggccgcgtcggtgcggaggccaggaggcggcgagagaagaggg

SEQ ID NO: 9119 - RNA, 5807 nt, Homo sapiens
  source 1..5807: mol_type = other RNA
actggacttggagtcagaaggcctaataatcagtccctaaaatcaagtggcaactactgatattgcaggatagtgcctaggaaagaattaagagacccaaagggttgaccttgcagagactccagcctatgaagtatcagcaagtgccaaaaatttatggctctgcaaaaaagcacagggtgactcaattatgcagagagctctaccacccaatgcaaaaccctggctcccggaatctaaaggacgaaatgttgcttaaagtatgatatattaacaattccagtgcttaaaagtttccctcactaaatatttctcttggatgtaccttagcaagctcttaggaagttgctgagtgttctgatgctggtcctgtgtcctttccactttctatcgtctacttcccagctcctgtgctttccttccagagagaactgtgtgtgcagtgtactttctatgcttcaccttcagggaccttctcttctttcctttctctgtctttgtccttgagctgtgttgtctgcactgctgaatggtggcagtcctgctgcaaggttgttgttcatagattgtatgacaccagcctcaacgggtgactgtgggaactagagttagaaatctgaagctcttctgcaaagtgccttgaactcttgatagggaagatgctattgaaagggacaaattcttttaaaagtaaatattgtggcagaagtctttgttgataaaatgacacaatgcagtaacagcttcagatctggggtaaaatcagatgccaatttccatctgaacacacgatgatcctgtgttgcatcattacacatttttacttcgtgtaaaaatttctaagcaaactaatactcaaaattaatgcaagtataatgaaagtttatcattcagatttattgccatataataaatctttcacaaaaatcaggaagaagcctctggtgactttgcagagctgaggcagtgatgcacgtggtggggcctccctcctgagcgggaaccaggactgggagcatcacttgcaggcctccatggaggctgctgccccagctgagctgttagctagtgagtgcttctactgtgtgatgaatgagaaaagggaaagaggggagggcaatcagggttctgggggcacctcagtgagcccagaggcctggaggagaggctgtatgattccccagtcaggccttccttgggagtgtgccctctgtcaagatgactgggtttttgaagggcctcatttcctcacacaacaagcactgacagtcctgcagcccagggactgtcctgtggcactgcccagccctcagactcagaggacagttctgtggtcctgccagaagctcagctgttccacatgacccttaaacatttaaacaattttttggtttaaaggaaaaggaagccaatcaaaatgctttggaaacaaattaaagttgcaaattatttccccacatagtaaatacatatccttgctacctgaaatgataatcatcactccccctgctggctgagagcgcttctcctccttcagactggctctgccacaaagctaagtattagtagaagttgttgccaagcctcacctctagcctgtacatgggctctgaggtgaacacaggagtcagagtccccactccagcagtgactggaggaggcctgacagaacaagccccttggggacaggaggcaagctgcactcacctctgggaccccacccgggatgggcgctccacgagtcccttggccttagggaacctctgtttcattccatccagacgaggatagggaagcttcctgccctacctcgacagcctctaagagcacagcttggccaggccttcccgtgtggagcccacacagtggtgcactgagaggctgccagtgttttgaccttttacagagcttggggtgactgagaatggttcctccgaggccctcggaagatttgatggactcaaataacacgggcctgcagccctgggacacaggacaggagaagccagccctgacacagatgagctggcagtggattcgaacagtgtgctcagtctcgtctgggcttttgtgctttctatgttgaagaccaaatactttttctttgagaatgaaactaggctccttatctagactgtgaaggggcccgtgaggacacagagtgtgactggaaaggaaggtcccaactggccctcaatgtggccccagtggctgtttccctgcaagaagctccttcctccagctcaggcaccaacacacggatcacaccggcccagaaacaaagagcaaaacatgcttttcatcccacgtggaatacagtatgaacaaattactctcctttttctattagtgtgggtgaaggaaaaagactgttttcaaatgaagcttttctttttcccaatgattaatacagagtagattaacttaatttgtgctagactccaatttaattccagcaacagttcacaggccatattcacagaaaagttaatctgggcttcatgagaagtagccattttctttttcttttctttctttttttttttttgcgagacagggtctcactttgtggctcaggctggagtgtactggcacgttcttagctcactgcagccttgaactcctgggctcaggcaatcctcctaccttagcctcctgagtagctaggactacaggaatgtgccatcatgcctggctaatttttaagttttttgtagagatgggatctcactatgttgcccaagctggtttcagattcctgtgctcaagggattctgctaacttggctccccaaagtgctgggattacaaatgtgagccactgtatctggcccatattcttttttaagaaaagatgcagaggtgttaaatattaatatcaaattgtccaggcatggtgtttatgaaattgtgtgccctctgacaggcaaccaaacacacacgacttcatttctttattaattcctgcctcatcatcttttctcattgatgctccttaatgtcaaaggaatctctctctctcacacacacataagaccaaaacaaatatcttgaacatgcaaaaaaatagtctacgcttttgaatagtgtgcactgttgaatagtgtgcactgttggatagtgtgcactgttgaagtgtgatgtgcctaaggcaacaggatcttgggaaagctctagatttttggcttcgaaataaaactgcatgttgaatagcaggtttttacatttattattgttgtgtatttcctcccctttttgcaatactatctacgctgagttatctattgccaactagcaccaattctccaaatcaaagtgtgtgaggaaaacacactcgtgcaatcctctttaacagaagatacaccaagtaacctgtctgtctacttctgttacccagaaataaaagaacttgaagggctgcttggctggaggggtccgggtgggagagcatcctgccctcagtcggaatccatggtgaacagctggatgtcctgtggattccagtacaggccgactgctgagttgtagacaagagaccagacataggggataaaaaactcctcgggctgctcctcttccacatatttgaatttcaattctggaaatttcttcagtctgtctttgggcagcgcaacgacgccttgcttaatgatttccaggacccgttccactgacagctcagctccagcttgcagcaaccttgagctaaagaaggagatcaccagatcaatattttgcattatatcctgaaatgaaggatgagttcgaaattgttcaaagagatcgcgtttgtaaagcagggcgtataccaagtttgggttgtggtgaagggaatttgtcaggcaggagttgatgatctctaacatcattcgaatcacttcttcaatgacatttaggtcttgtgcataatctggtagaggaacatcattagaactcagcgaacctctcaaggactgtgtggcttgttccagaactttgttgtgttttttagacagcaaagaaaataaactggaagcataggatctgagaatgtgagagcaagttaaagacaagagttcctctccattgtcactgagggtcgagaagcaatgctgaagcgtagaacagtgagagtgggggaaatacagtttgtccaacacataaacatatctccgcaagtggcggcaggtataactgatgatcctctgggcagcatactgatggagagaacgaaactgtgccgacatatttgctaaagctgccaaacaatttgtgtgaaggtacttgtctcgtgtcctagtcatgttgtattgaatggttcttattaccaccaggatcaggagactccccaaggagatttcagttaaaactcgttctgaataccaagtaatattttttagtatcacttcatgaatggatctgttgaagccatcatcttccgtaaggatcaacaatattataagggccatatacacatggtgtgaattcctttcttcaacatgatacagaatctcaagaattggtaaaacaagattttccatatctgtgcgagccaacatgtatgttctaatattactattttgatggagcaaggtatacaagaggagagttgcttgatcagatgtctgctgttcacaaagagctgtgtacaaactattaaagttgatctggaaggcatgtggaattgatgaggggaaaggactgctatcttgtgtgttcttgaaggacataatggcttgtctgtaggggtttggcgcatctgaggcatctgtcagattggccaacaccagcagaagcaggagactctggttggccagaggggaagaaagctctggagaggcagccgctttgctgcccacaccacctagtgtgaagacagtccagagtcctgttgctactcctgatgcaagtccataaagcagtcctcccccatccgactgctgagggaaaacatgggcccctggaggaggtggcttttcttgtctgataaagttatataataaggtcttcacaagtttgctggtgtatggaagaaagagtggaatatcagtgatcaactgcatcaaacagcacagcaattcttccaaaagatcttctgagtcagaactgtaattgccaggagatttttcttcataagtaaaatgaagttgtaattcctcctctgacatctgacagatgaacactttcagcaaacagcaaataataaacaaagcattgtgtgtctgccaaatgaagatgtggttctgacattctgctgaaagttttagttctttggttctagaaaggaagaccttaattagtgcaccaagatttcctgttcgaggattgttttcaactaatgacctgcagactgaaatggttgcttcctccaagagtttcaactcactactgctagttggtgcagggaaagaaaatgagagaagctgattccagaacgggtcattctcagagatagattccgtgcctgataactttttcaagtactcatttttaggaagatcgccgattctgctgctattcgatcccatcttctagcttaagcagataatttgtccttaaacctgcatttccaaaagacaacctgtctcagccggctgggggatctgctccagctccacggacccgcggacggatgggagggtggcagaggggtcaggagaagtcgctgtcgccgccgcagcccaggtggcgcacaccggctcaggcctccatgtttccacgtctcagcgggtacagatccggctccggtccggcctgcagctcggccccggctcggctccagcccgggccgcgtcggtgcggaggccaggaggcggcgagagaagaggg

SEQ ID NO: 9120 - RNA, 6191 nt, Homo sapiens
  source 1..6191: mol_type = other RNA
actggacttggagtcagaaggcctaataatcagtccctaaaatcaagtggcaactactgatattgcaggatagtgcctaggaaagaattaagagacccaaagggttgaccttgcagagactccagcctatgaagtatcagcaagtgccaaaaatttatggctctgcaaaaaagcacagggtgactcaattatgcagagagctctaccacccaatgcaaaaccctggctcccggaatctaaaggacgaaatgttgcttaaagtatgatatattaacaattccagtgcttaaaagtttccctcactaaatatttctcttggatgtaccttagcaagctcttaggaagttgctgagtgttctgatgctggtcctgtgtcctttccactttctatcgtctacttcccagctcctgtgctttccttccagagagaactgtgtgtgcagtgtactttctatgcttcaccttcagggaccttctcttctttcctttctctgtctttgtccttgagctgtgttgtctgcactgctgaatggtggcagtcctgctgcaaggttgttgttcatagattgtatgacaccagcctcaacgggtgactgtgggaactagagttagaaatctgaagctcttctgcaaagtgccttgaactcttgatagggaagatgctattgaaagggacaaattcttttaaaagtaaatattgtggcagaagtctttgttgataaaatgacacaatgcagtaacagcttcagatctggggtaaaatcagatgccaatttccatctgaacacacgatgatcctgtgttgcatcattacacatttttacttcgtgtaaaaatttctaagcaaactaatactcaaaattaatgcaagtataatgaaagtttatcattcagatttattgccatataataaatctttcacaaaaatcaggaagaagcctctggtgactttgcagagctgaggcagtgatgcacgtggtggggcctccctcctgagcgggaaccaggactgggagcatcacttgcaggcctccatggaggctgctgccccagctgagctgttagctagtgagtgcttctactgtgtgatgaatgagaaaagggaaagaggggagggcaatcagggttctgggggcacctcagtgagcccagaggcctggaggagaggctgtatgattccccagtcaggccttccttgggagtgtgccctctgtcaagatgactgggtttttgaagggcctcatttcctcacacaacaagcactgacagtcctgcagcccagggactgtcctgtggcactgcccagccctcagactcagaggacagttctgtggtcctgccagaagctcagctgttccacatgacccttaaacatttaaacaattttttggtttaaaggaaaaggaagccaatcaaaatgctttggaaacaaattaaagttgcaaattatttccccacatagtaaatacatatccttgctacctgaaatgataatcatcactccccctgctggctgagagcgcttctcctccttcagactggctctgccacaaagctaagtattagtagaagttgttgccaagcctcacctctagcctgtacatgggctctgaggtgaacacaggagtcagagtccccactccagcagtgactggaggaggcctgacagaacaagccccttggggacaggaggcaagctgcactcacctctgggaccccacccgggatgggcgctccacgagtcccttggccttagggaacctctgtttcattccatccagacgaggatagggaagcttcctgccctacctcgacagcctctaagagcacagcttggccaggccttcccgtgtggagcccacacagtggtgcactgagaggctgccagtgttttgaccttttacagagcttggggtgactgagaatggttcctccgaggccctcggaagatttgatggactcaaataacacgggcctgcagccctgggacacaggacaggagaagccagccctgacacagatgagctggcagtggattcgaacagtgtgctcagtctcgtctgggcttttgtgctttctatgttgaagaccaaatactttttctttgagaatgaaactaggctccttatctagactgtgaaggggcccgtgaggacacagagtgtgactggaaaggaaggtcccaactggccctcaatgtggccccagtggctgtttccctgcaagaagctccttcctccagctcaggcaccaacacacggatcacaccggcccagaaacaaagagcaaaacatgcttttcatcccacgtggaatacagtatgaacaaattactctcctttttctattagtgtgggtgaaggaaaaagactgttttcaaatgaagcttttctttttcccaatgattaatacagagtagattaacttaatttgtgctagactccaatttaattccagcaacagttcacaggccatattcacagaaaagttaatctgggcttcatgagaagtagccattttctttttcttttctttctttttttttttttgcgagacagggtctcactttgtggctcaggctggagtgtactggcacgttcttagctcactgcagccttgaactcctgggctcaggcaatcctcctaccttagcctcctgagtagctaggactacaggaatgtgccatcatgcctggctaatttttaagttttttgtagagatgggatctcactatgttgcccaagctggtttcagattcctgtgctcaagggattctgctaacttggctccccaaagtgctgggattacaaatgtgagccactgtatctggcccatattcttttttaagaaaagatgcagaggtgttaaatattaatatcaaattgtccaggcatggtgtttatgaaattgtgtgccctctgacaggcaaccaaacacacacgacttcatttctttattaattcctgcctcatcatcttttctcattgatgctccttaatgtcaaaggaatctctctctctcacacacacataagaccaaaacaaatatcttgaacatgcaaaaaaatagtctacgcttttgaatagtgtgcactgttgaatagtgtgcactgttggatagtgtgcactgttgaagtgtgatgtgcctaaggcaacaggatcttgggaaagctctagatttttggcttcgaaataaaactgcatgttgaatagcaggtttttacatttattattgttgtgtatttcctcccctttttgcaatactatctacgctgagttatctattgccaactagcaccaattctccaaatcaaagtgtgtgaggaaaacacactcgtgcaatcctctttaacagaagatacaccaagtaacctgtctgtctacttctgttacccagaaataaaagaacttgaagggctgcttggctggaggggtccgggtgggagagcatcctgccctcagtcggaatccatggtgaacagctggatgtcctgtggattccagtacaggccgactgctgagttgtagacaagagaccagacataggggataaaaaactcctcgggctgctcctcttccacatatttgaatttcaattctggaaatttcttcagtctgtctttgggcagcgcaacgacgccttgcttaatgatttccaggacccgttccactgacagctcagctccagcttgcagcaaccttgagctaaagaaggagatcaccagatcaatattttgcattatatcctgaaatgaaggatgagttcgaaattgttcaaagagatcgcgtttgtaaagcagggcgtataccaagtttgggttgtggtgaagggaatttgtcaggcaggagttgatgatctctaacatcattcgaatcacttcttcaatgacatttaggtcttgtgcataatctggtagaggaacatcattagaactcagcgaacctctcaaggactgtgtggcttgttccagaactttgttgtgttttttagacagcaaagaaaataaactggaagcataggatctgagaatgtgagagcaagttaaagacaagagttcctctccattgtcactgagggtcgagaagcaatgctgaagcgtagaacagtgagagtgggggaaatacagtttgtccaacacataaacatatctccgcaagtggcggcaggtataactgatgatcctctgggcagcatactgatggagagaacgaaactgtgccgacatatttgctaaagctgccaaacaatttgtgtgaaggtacttgtctcgtgtcctagtcatgttgtattgaatggttcttattaccaccaggatcaggagactccccaaggagatttcagttaaaactcgttctgaataccaagtaatattttttagtatcacttcatgaatggatctgttgaagccatcatcttccgtaaggatcaacaatattataagggccatatacacatggtgtgaattcctttcttcaacatgatacagaatctcaagaattggtaaaacaagattttccatatctgtgcgagccaacatgtatgttctaatattactattttgatggagcaaggtatacaagaggagagttgcttgatcagatgtctgctgttcacaaagagctgtgtacaaactattaaagttgatctggaaggcatgtggaattgatgaggggaaaggactgctatcttgtgtgttcttgaaggacataatggcttgtctgtaggggtttggcgcatctgaggcatctgtcagattggccaacaccagcagaagcaggagactctggttggccagaggggaagaaagctctggagaggcagccgctttgctgcccacaccacctagtgtgaagacagtccagagtcctgttgctactcctgatgcaagtccataaagcagtcctcccccatccgactgctgagggaaaacatgggcccctggaggaggtggcttttcttgtctgataaagttatataataaggtcttcacaagtttgctggtgtatggaagacatggacctcgcatcaaatacttgtggctgatgctctgtcgcaaaacttctttgtggaagagttggcaggaaaggaaaacaaccattgttgatatagcttctactgatatttcatatgtaatatctaagagtggaatatcagtgatcaactgcatcaaacagcacagcaattcttccaaaagatcttctgagtcagaactgtaattgccaggagatttttcttcataagtaaaatgaagttgtaattcctcctctgacatctgacagatgaacactttcagcaaacagcaaataataaacaaagcattgtgtgtctgccaaatgaagatgtggttctgacattctgctgaaagttttagttctttggttctagaaaggaagaccttaattagtgcaccaagatttcctgttcgaggattgttttcaactaatgacctgcagactgaaatggttgcttcctccaagagtttcaactcactactgctagttggtgcagggaaagaaaatgagagaagctgattccagaacgggtcattctcagagatagattccgtgcctgataactttttcaagtactcatttttaggaagatcgccgattctgctgctattcgatcccatcttctagcttaagcagataatttgtccttaaacctgcatttccaaaagacaacctctacaggaaatgcccaatggaggtgatgtcactagggttcaagttccctcctctttgcaagaccttaggcaaataaaggtgactgaggccaattttctgaagaccctgataggtatatagaagctttccaaaatttaactcaggtgtttcacctctcatgaagagattttatgttgcttctaagccaaaccctaattacagctgaagagcaggcagcaaagaaattgaaagataagcaacgtttcctatagtaggcctgtctcagccggctgggggatctgctccagctccacggacccgcggacggatgggagggtggcagaggggtcaggagaagtcgctgtcgccgccgcagcccaggtggcgcacaccggctcaggcctccatgtttccacgtctcagcgggtacagatccggctccggtccggcctgcagctcggccccggctcggctccagcccgggccgcgtcggtgcggaggccaggaggcggcgagagaagaggg

SEQ ID NO: 9121 - RNA, 5933 nt, Homo sapiens
  source 1..5933: mol_type = other RNA
actggacttggagtcagaaggcctaataatcagtccctaaaatcaagtggcaactactgatattgcaggatagtgcctaggaaagaattaagagacccaaagggttgaccttgcagagactccagcctatgaagtatcagcaagtgccaaaaatttatggctctgcaaaaaagcacagggtgactcaattatgcagagagctctaccacccaatgcaaaaccctggctcccggaatctaaaggacgaaatgttgcttaaagtatgatatattaacaattccagtgcttaaaagtttccctcactaaatatttctcttggatgtaccttagcaagctcttaggaagttgctgagtgttctgatgctggtcctgtgtcctttccactttctatcgtctacttcccagctcctgtgctttccttccagagagaactgtgtgtgcagtgtactttctatgcttcaccttcagggaccttctcttctttcctttctctgtctttgtccttgagctgtgttgtctgcactgctgaatggtggcagtcctgctgcaaggttgttgttcatagattgtatgacaccagcctcaacgggtgactgtgggaactagagttagaaatctgaagctcttctgcaaagtgccttgaactcttgatagggaagatgctattgaaagggacaaattcttttaaaagtaaatattgtggcagaagtctttgttgataaaatgacacaatgcagtaacagcttcagatctggggtaaaatcagatgccaatttccatctgaacacacgatgatcctgtgttgcatcattacacatttttacttcgtgtaaaaatttctaagcaaactaatactcaaaattaatgcaagtataatgaaagtttatcattcagatttattgccatataataaatctttcacaaaaatcaggaagaagcctctggtgactttgcagagctgaggcagtgatgcacgtggtggggcctccctcctgagcgggaaccaggactgggagcatcacttgcaggcctccatggaggctgctgccccagctgagctgttagctagtgagtgcttctactgtgtgatgaatgagaaaagggaaagaggggagggcaatcagggttctgggggcacctcagtgagcccagaggcctggaggagaggctgtatgattccccagtcaggccttccttgggagtgtgccctctgtcaagatgactgggtttttgaagggcctcatttcctcacacaacaagcactgacagtcctgcagcccagggactgtcctgtggcactgcccagccctcagactcagaggacagttctgtggtcctgccagaagctcagctgttccacatgacccttaaacatttaaacaattttttggtttaaaggaaaaggaagccaatcaaaatgctttggaaacaaattaaagttgcaaattatttccccacatagtaaatacatatccttgctacctgaaatgataatcatcactccccctgctggctgagagcgcttctcctccttcagactggctctgccacaaagctaagtattagtagaagttgttgccaagcctcacctctagcctgtacatgggctctgaggtgaacacaggagtcagagtccccactccagcagtgactggaggaggcctgacagaacaagccccttggggacaggaggcaagctgcactcacctctgggaccccacccgggatgggcgctccacgagtcccttggccttagggaacctctgtttcattccatccagacgaggatagggaagcttcctgccctacctcgacagcctctaagagcacagcttggccaggccttcccgtgtggagcccacacagtggtgcactgagaggctgccagtgttttgaccttttacagagcttggggtgactgagaatggttcctccgaggccctcggaagatttgatggactcaaataacacgggcctgcagccctgggacacaggacaggagaagccagccctgacacagatgagctggcagtggattcgaacagtgtgctcagtctcgtctgggcttttgtgctttctatgttgaagaccaaatactttttctttgagaatgaaactaggctccttatctagactgtgaaggggcccgtgaggacacagagtgtgactggaaaggaaggtcccaactggccctcaatgtggccccagtggctgtttccctgcaagaagctccttcctccagctcaggcaccaacacacggatcacaccggcccagaaacaaagagcaaaacatgcttttcatcccacgtggaatacagtatgaacaaattactctcctttttctattagtgtgggtgaaggaaaaagactgttttcaaatgaagcttttctttttcccaatgattaatacagagtagattaacttaatttgtgctagactccaatttaattccagcaacagttcacaggccatattcacagaaaagttaatctgggcttcatgagaagtagccattttctttttcttttctttctttttttttttttgcgagacagggtctcactttgtggctcaggctggagtgtactggcacgttcttagctcactgcagccttgaactcctgggctcaggcaatcctcctaccttagcctcctgagtagctaggactacaggaatgtgccatcatgcctggctaatttttaagttttttgtagagatgggatctcactatgttgcccaagctggtttcagattcctgtgctcaagggattctgctaacttggctccccaaagtgctgggattacaaatgtgagccactgtatctggcccatattcttttttaagaaaagatgcagaggtgttaaatattaatatcaaattgtccaggcatggtgtttatgaaattgtgtgccctctgacaggcaaccaaacacacacgacttcatttctttattaattcctgcctcatcatcttttctcattgatgctccttaatgtcaaaggaatctctctctctcacacacacataagaccaaaacaaatatcttgaacatgcaaaaaaatagtctacgcttttgaatagtgtgcactgttgaatagtgtgcactgttggatagtgtgcactgttgaagtgtgatgtgcctaaggcaacaggatcttgggaaagctctagatttttggcttcgaaataaaactgcatgttgaatagcaggtttttacatttattattgttgtgtatttcctcccctttttgcaatactatctacgctgagttatctattgccaactagcaccaattctccaaatcaaagtgtgtgaggaaaacacactcgtgcaatcctctttaacagaagatacaccaagtaacctgtctgtctacttctgttacccagaaataaaagaacttgaagggctgcttggctggaggggtccgggtgggagagcatcctgccctcagtcggaatccatggtgaacagctggatgtcctgtggattccagtacaggccgactgctgagttgtagacaagagaccagacataggggataaaaaactcctcgggctgctcctcttccacatatttgaatttcaattctggaaatttcttcagtctgtctttgggcagcgcaacgacgccttgcttaatgatttccaggacccgttccactgacagctcagctccagcttgcagcaaccttgagctaaagaaggagatcaccagatcaatattttgcattatatcctgaaatgaaggatgagttcgaaattgttcaaagagatcgcgtttgtaaagcagggcgtataccaagtttgggttgtggtgaagggaatttgtcaggcaggagttgatgatctctaacatcattcgaatcacttcttcaatgacatttaggtcttgtgcataatctggtagaggaacatcattagaactcagcgaacctctcaaggactgtgtggcttgttccagaactttgttgtgttttttagacagcaaagaaaataaactggaagcataggatctgagaatgtgagagcaagttaaagacaagagttcctctccattgtcactgagggtcgagaagcaatgctgaagcgtagaacagtgagagtgggggaaatacagtttgtccaacacataaacatatctccgcaagtggcggcaggtataactgatgatcctctgggcagcatactgatggagagaacgaaactgtgccgacatatttgctaaagctgccaaacaatttgtgtgaaggtacttgtctcgtgtcctagtcatgttgtattgaatggttcttattaccaccaggatcaggagactccccaaggagatttcagttaaaactcgttctgaataccaagtaatattttttagtatcacttcatgaatggatctgttgaagccatcatcttccgtaaggatcaacaatattataagggccatatacacatggtgtgaattcctttcttcaacatgatacagaatctcaagaattggtaaaacaagattttccatatctgtgcgagccaacatgtatgttctaatattactattttgatggagcaaggtatacaagaggagagttgcttgatcagatgtctgctgttcacaaagagctgtgtacaaactattaaagttgatctggaaggcatgtggaattgatgaggggaaaggactgctatcttgtgtgttcttgaaggacataatggcttgtctgtaggggtttggcgcatctgaggcatctgtcagattggccaacaccagcagaagcaggagactctggttggccagaggggaagaaagctctggagaggcagccgctttgctgcccacaccacctagtgtgaagacagtccagagtcctgttgctactcctgatgcaagtccataaagcagtcctcccccatccgactgctgagggaaaacatgggcccctggaggaggtggcttttcttgtctgataaagttatataataaggtcttcacaagtttgctggtgtatggaagacatggacctcgcatcaaatacttgtggctgatgctctgtcgcaaaacttctttgtggaagagttggcaggaaaggaaaacaaccattgttgatatagcttctactgatatttcatatgtaatatctaagagtggaatatcagtgatcaactgcatcaaacagcacagcaattcttccaaaagatcttctgagtcagaactgtaattgccaggagatttttcttcataagtaaaatgaagttgtaattcctcctctgacatctgacagatgaacactttcagcaaacagcaaataataaacaaagcattgtgtgtctgccaaatgaagatgtggttctgacattctgctgaaagttttagttctttggttctagaaaggaagaccttaattagtgcaccaagatttcctgttcgaggattgttttcaactaatgacctgcagactgaaatggttgcttcctccaagagtttcaactcactactgctagttggtgcagggaaagaaaatgagagaagctgattccagaacgggtcattctcagagatagattccgtgcctgataactttttcaagtactcatttttaggaagatcgccgattctgctgctattcgatcccatcttctagcttaagcagataatttgtccttaaacctgcatttccaaaagacaacctgtctcagccggctgggggatctgctccagctccacggacccgcggacggatgggagggtggcagaggggtcaggagaagtcgctgtcgccgccgcagcccaggtggcgcacaccggctcaggcctccatgtttccacgtctcagcgggtacagatccggctccggtccggcctgcagctcggccccggctcggctccagcccgggccgcgtcggtgcggaggccaggaggcggcgagagaagaggg

SEQ ID NO: 9122 - RNA, 5930 nt, Homo sapiens
  source 1..5930: mol_type = other RNA
actggacttggagtcagaaggcctaataatcagtccctaaaatcaagtggcaactactgatattgcaggatagtgcctaggaaagaattaagagacccaaagggttgaccttgcagagactccagcctatgaagtatcagcaagtgccaaaaatttatggctctgcaaaaaagcacagggtgactcaattatgcagagagctctaccacccaatgcaaaaccctggctcccggaatctaaaggacgaaatgttgcttaaagtatgatatattaacaattccagtgcttaaaagtttccctcactaaatatttctcttggatgtaccttagcaagctcttaggaagttgctgagtgttctgatgctggtcctgtgtcctttccactttctatcgtctacttcccagctcctgtgctttccttccagagagaactgtgtgtgcagtgtactttctatgcttcaccttcagggaccttctcttctttcctttctctgtctttgtccttgagctgtgttgtctgcactgctgaatggtggcagtcctgctgcaaggttgttgttcatagattgtatgacaccagcctcaacgggtgactgtgggaactagagttagaaatctgaagctcttctgcaaagtgccttgaactcttgatagggaagatgctattgaaagggacaaattcttttaaaagtaaatattgtggcagaagtctttgttgataaaatgacacaatgcagtaacagcttcagatctggggtaaaatcagatgccaatttccatctgaacacacgatgatcctgtgttgcatcattacacatttttacttcgtgtaaaaatttctaagcaaactaatactcaaaattaatgcaagtataatgaaagtttatcattcagatttattgccatataataaatctttcacaaaaatcaggaagaagcctctggtgactttgcagagctgaggcagtgatgcacgtggtggggcctccctcctgagcgggaaccaggactgggagcatcacttgcaggcctccatggaggctgctgccccagctgagctgttagctagtgagtgcttctactgtgtgatgaatgagaaaagggaaagaggggagggcaatcagggttctgggggcacctcagtgagcccagaggcctggaggagaggctgtatgattccccagtcaggccttccttgggagtgtgccctctgtcaagatgactgggtttttgaagggcctcatttcctcacacaacaagcactgacagtcctgcagcccagggactgtcctgtggcactgcccagccctcagactcagaggacagttctgtggtcctgccagaagctcagctgttccacatgacccttaaacatttaaacaattttttggtttaaaggaaaaggaagccaatcaaaatgctttggaaacaaattaaagttgcaaattatttccccacatagtaaatacatatccttgctacctgaaatgataatcatcactccccctgctggctgagagcgcttctcctccttcagactggctctgccacaaagctaagtattagtagaagttgttgccaagcctcacctctagcctgtacatgggctctgaggtgaacacaggagtcagagtccccactccagcagtgactggaggaggcctgacagaacaagccccttggggacaggaggcaagctgcactcacctctgggaccccacccgggatgggcgctccacgagtcccttggccttagggaacctctgtttcattccatccagacgaggatagggaagcttcctgccctacctcgacagcctctaagagcacagcttggccaggccttcccgtgtggagcccacacagtggtgcactgagaggctgccagtgttttgaccttttacagagcttggggtgactgagaatggttcctccgaggccctcggaagatttgatggactcaaataacacgggcctgcagccctgggacacaggacaggagaagccagccctgacacagatgagctggcagtggattcgaacagtgtgctcagtctcgtctgggcttttgtgctttctatgttgaagaccaaatactttttctttgagaatgaaactaggctccttatctagactgtgaaggggcccgtgaggacacagagtgtgactggaaaggaaggtcccaactggccctcaatgtggccccagtggctgtttccctgcaagaagctccttcctccagctcaggcaccaacacacggatcacaccggcccagaaacaaagagcaaaacatgcttttcatcccacgtggaatacagtatgaacaaattactctcctttttctattagtgtgggtgaaggaaaaagactgttttcaaatgaagcttttctttttcccaatgattaatacagagtagattaacttaatttgtgctagactccaatttaattccagcaacagttcacaggccatattcacagaaaagttaatctgggcttcatgagaagtagccattttctttttcttttctttctttttttttttttgcgagacagggtctcactttgtggctcaggctggagtgtactggcacgttcttagctcactgcagccttgaactcctgggctcaggcaatcctcctaccttagcctcctgagtagctaggactacaggaatgtgccatcatgcctggctaatttttaagttttttgtagagatgggatctcactatgttgcccaagctggtttcagattcctgtgctcaagggattctgctaacttggctccccaaagtgctgggattacaaatgtgagccactgtatctggcccatattcttttttaagaaaagatgcagaggtgttaaatattaatatcaaattgtccaggcatggtgtttatgaaattgtgtgccctctgacaggcaaccaaacacacacgacttcatttctttattaattcctgcctcatcatcttttctcattgatgctccttaatgtcaaaggaatctctctctctcacacacacataagaccaaaacaaatatcttgaacatgcaaaaaaatagtctacgcttttgaatagtgtgcactgttgaatagtgtgcactgttggatagtgtgcactgttgaagtgtgatgtgcctaaggcaacaggatcttgggaaagctctagatttttggcttcgaaataaaactgcatgttgaatagcaggtttttacatttattattgttgtgtatttcctcccctttttgcaatactatctacgctgagttatctattgccaactagcaccaattctccaaatcaaagtgtgtgaggaaaacacactcgtgcaatcctctttaacagaagatacaccaagtaacctgtctgtctacttctgttacccagaaataaaagaacttgaagggctgcttggctggaggggtccgggtgggagagcatcctgccctcagtcggaatccatggtgaacagctggatgtcctgtggattccagtacaggccgactgctgagttgtagacaagagaccagacataggggataaaaaactcctcgggctgctcctcttccacatatttgaatttcaattctggaaatttcttcagtctgtctttgggcagcgcaacgacgccttgcttaatgatttccaggacccgttccactgacagctcagctccagcttgcagcaaccttgagctaaagaaggagatcaccagatcaatattttgcattatatcctgaaatgaaggatgagttcgaaattgttcaaagagatcgcgtttgtaaagcagggcgtataccaagtttgggttgtggtgaagggaatttgtcaggcaggagttgatgatctctaacatcattcgaatcacttcttcaatgacatttaggtcttgtgcataatctggtagaggaacatcattagaactcagcgaacctctcaaggactgtgtggcttgttccagaactttgttgtgttttttagacagcaaagaaaataaactggaagcataggatctgagaatgtgagagcaagttaaagacaagagttcctctccattgtcactgagggtcgagaagcaatgctgaagcgtagaacagtgagagtgggggaaatacagtttgtccaacacataaacatatctccgcaagtggcggcaggtataactgatgatcctctgggcagcatactgatggagagaacgaaactgtgccgacatatttgctaaagctgccaaacaatttgtgtgaaggtacttgtctcgtgtcctagtcatgttgtattgaatggttcttattaccaccaggatcaggagactccccaaggagatttcagttaaaactcgttctgaataccaagtaatattttttagtatcacttcatgaatggatctgttgaagccatcatcttccgtaaggatcaacaatattataagggccatatacacatggtgtgaattcctttcttcaacatgatacagaatctcaagaattggtaaaacaagattttccatatctgtgcgagccaacatgtatgttctaatattactattttgatggagcaaggtatacaagaggagagttgcttgatcagatgtctgctgttcacaaagagctgtgtacaaactattaaagttgatctggaaggcatgtggaattgatgaggggaaaggactgctatcttgtgtgttcttgaaggacataatggcttgtctgtaggggtttggcgcatctgaggcatctgtcagattggccaacaccagcagaagcaggagactctggttggccagaggggaagaaagctctggagaggcagccgctttgctgcccacaccacctagtgtgaagacagtccagagtcctgttgctactcctgatgcaagtccataaagcagtcctcccccatccgactgctgagggaaaacatgggcccctggaggaggtggcttttcttgtctgataaagttatataataaggtcttcacaagtttgctggtgtatggaagacatggacctcgcatcaaatacttgtggctgatgctctgtcgcaaaacttctttgtggaagagttggcaggaaaggaaaacaaccattgttgatatagcttctactgatatttcatatgtaatatctaagagtggaatatcagtgatcaactgcatcaaacagcacagcaattcttccaaaagatcttctgagtcagaactgtaattgccaggagatttttcttcataagtaaaatgaagttgtaattcctcctctgacatctgacagatgaacactttcagcaaacagcaaataataaacaaagcattgtgtgtctgccaaatgaagatgtggttctgacattctgctgaaagttttagttctttggttctagaaaggaagaccttaattagtgcaccaagatttcctgttcgaggattgttttcaactaatgacctgcagactgaaatggttgcttcctccaagagtttcaactcactgctagttggtgcagggaaagaaaatgagagaagctgattccagaacgggtcattctcagagatagattccgtgcctgataactttttcaagtactcatttttaggaagatcgccgattctgctgctattcgatcccatcttctagcttaagcagataatttgtccttaaacctgcatttccaaaagacaacctgtctcagccggctgggggatctgctccagctccacggacccgcggacggatgggagggtggcagaggggtcaggagaagtcgctgtcgccgccgcagcccaggtggcgcacaccggctcaggcctccatgtttccacgtctcagcgggtacagatccggctccggtccggcctgcagctcggccccggctcggctccagcccgggccgcgtcggtgcggaggccaggaggcggcgagagaagaggg

SEQ ID NO: 9123 - RNA, 5930 nt, Homo sapiens
  source 1..5930: mol_type = other RNA
actggacttggagtcagaaggcctaataatcagtccctaaaatcaagtggcaactactgatattgcaggatagtgcctaggaaagaattaagagacccaaagggttgaccttgcagagactccagcctatgaagtatcagcaagtgccaaaaatttatggctctgcaaaaaagcacagggtgactcaattatgcagagagctctaccacccaatgcaaaaccctggctcccggaatctaaaggacgaaatgttgcttaaagtatgatatattaacaattccagtgcttaaaagtttccctcactaaatatttctcttggatgtaccttagcaagctcttaggaagttgctgagtgttctgatgctggtcctgtgtcctttccactttctatcgtctacttcccagctcctgtgctttccttccagagagaactgtgtgtgcagtgtactttctatgcttcaccttcagggaccttctcttctttcctttctctgtctttgtccttgagctgtgttgtctgcactgctgaatggtggcagtcctgctgcaaggttgttgttcatagattgtatgacaccagcctcaacgggtgactgtgggaactagagttagaaatctgaagctcttctgcaaagtgccttgaactcttgatagggaagatgctattgaaagggacaaattcttttaaaagtaaatattgtggcagaagtctttgttgataaaatgacacaatgcagtaacagcttcagatctggggtaaaatcagatgccaatttccatctgaacacacgatgatcctgtgttgcatcattacacatttttacttcgtgtaaaaatttctaagcaaactaatactcaaaattaatgcaagtataatgaaagtttatcattcagatttattgccatataataaatctttcacaaaaatcaggaagaagcctctggtgactttgcagagctgaggcagtgatgcacgtggtggggcctccctcctgagcgggaaccaggactgggagcatcacttgcaggcctccatggaggctgctgccccagctgagctgttagctagtgagtgcttctactgtgtgatgaatgagaaaagggaaagaggggagggcaatcagggttctgggggcacctcagtgagcccagaggcctggaggagaggctgtatgattccccagtcaggccttccttgggagtgtgccctctgtcaagatgactgggtttttgaagggcctcatttcctcacacaacaagcactgacagtcctgcagcccagggactgtcctgtggcactgcccagccctcagactcagaggacagttctgtggtcctgccagaagctcagctgttccacatgacccttaaacatttaaacaattttttggtttaaaggaaaaggaagccaatcaaaatgctttggaaacaaattaaagttgcaaattatttccccacatagtaaatacatatccttgctacctgaaatgataatcatcactccccctgctggctgagagcgcttctcctccttcagactggctctgccacaaagctaagtattagtagaagttgttgccaagcctcacctctagcctgtacatgggctctgaggtgaacacaggagtcagagtccccactccagcagtgactggaggaggcctgacagaacaagccccttggggacaggaggcaagctgcactcacctctgggaccccacccgggatgggcgctccacgagtcccttggccttagggaacctctgtttcattccatccagacgaggatagggaagcttcctgccctacctcgacagcctctaagagcacagcttggccaggccttcccgtgtggagcccacacagtggtgcactgagaggctgccagtgttttgaccttttacagagcttggggtgactgagaatggttcctccgaggccctcggaagatttgatggactcaaataacacgggcctgcagccctgggacacaggacaggagaagccagccctgacacagatgagctggcagtggattcgaacagtgtgctcagtctcgtctgggcttttgtgctttctatgttgaagaccaaatactttttctttgagaatgaaactaggctccttatctagactgtgaaggggcccgtgaggacacagagtgtgactggaaaggaaggtcccaactggccctcaatgtggccccagtggctgtttccctgcaagaagctccttcctccagctcaggcaccaacacacggatcacaccggcccagaaacaaagagcaaaacatgcttttcatcccacgtggaatacagtatgaacaaattactctcctttttctattagtgtgggtgaaggaaaaagactgttttcaaatgaagcttttctttttcccaatgattaatacagagtagattaacttaatttgtgctagactccaatttaattccagcaacagttcacaggccatattcacagaaaagttaatctgggcttcatgagaagtagccattttctttttcttttctttctttttttttttttgcgagacagggtctcactttgtggctcaggctggagtgtactggcacgttcttagctcactgcagccttgaactcctgggctcaggcaatcctcctaccttagcctcctgagtagctaggactacaggaatgtgccatcatgcctggctaatttttaagttttttgtagagatgggatctcactatgttgcccaagctggtttcagattcctgtgctcaagggattctgctaacttggctccccaaagtgctgggattacaaatgtgagccactgtatctggcccatattcttttttaagaaaagatgcagaggtgttaaatattaatatcaaattgtccaggcatggtgtttatgaaattgtgtgccctctgacaggcaaccaaacacacacgacttcatttctttattaattcctgcctcatcatcttttctcattgatgctccttaatgtcaaaggaatctctctctctcacacacacataagaccaaaacaaatatcttgaacatgcaaaaaaatagtctacgcttttgaatagtgtgcactgttgaatagtgtgcactgttggatagtgtgcactgttgaagtgtgatgtgcctaaggcaacaggatcttgggaaagctctagatttttggcttcgaaataaaactgcatgttgaatagcaggtttttacatttattattgttgtgtatttcctcccctttttgcaatactatctacgctgagttatctattgccaactagcaccaattctccaaatcaaagtgtgtgaggaaaacacactcgtgcaatcctctttaacagaagatacaccaagtaacctgtctgtctacttctgttacccagaaataaaagaacttgaagggctgcttggctggaggggtccgggtgggagagcatcctgccctcagtcggaatccatggtgaacagctggatgtcctgtggattccagtacaggccgactgctgagttgtagacaagagaccagacataggggataaaaaactcctcgggctgctcctcttccacatatttgaatttcaattctggaaatttcttcagtctgtctttgggcagcgcaacgacgccttgcttaatgatttccaggacccgttccactgacagctcagctccagcttgcagcaaccttgagctaaagaaggagatcaccagatcaatattttgcattatatcctgaaatgaaggatgagttcgaaattgttcaaagagatcgcgtttgtaaagcagggcgtataccaagtttgggttgtggtgaagggaatttgtcaggcaggagttgatgatctctaacatcattcgaatcacttcttcaatgacatttaggtcttgtgcataatctggtagaggaacatcattagaactcagcgaacctctcaaggactgtgtggcttgttccagaactttgttgtgttttttagacagcaaagaaaataaactggaagcataggatctgagaatgtgagagcaagttaaagacaagagttcctctccattgtcactgagggtcgagaagcaatgctgaagcgtagaacagtgagagtgggggaaatacagtttgtccaacacataaacatatctccgcaagtggcggcaggtataactgatgatcctctgggcagcatactgatggagagaacgaaactgtgccgacatatttgctaaagctgccaaacaatttgtgtgaaggtacttgtctcgtgtcctagtcatgttgtattgaatggttcttattaccaccaggatcaggagactccccaaggagatttcagttaaaactcgttctgaataccaagtaatattttttagtatcacttcatgaatggatctgttgaagccatcatcttccgtaaggatcaacaatattataagggccatatacacatggtgtgaattcctttcttcaacatgatacagaatctcaagaattggtaaaacaagattttccatatctgtgcgagccaacatgtatgttctaatattactattttgatggagcaaggtatacaagaggagagttgcttgatcagatgtctgctgttcacaaagagctgtgtacaaactattaaagttgatctggaaggcatgtggaattgatgaggggaaaggactgctatcttgtgtgttcttgaaggacataatggcttgtctgtaggggtttggcgcatctgaggcatctgtcagattggccaacaccagcagaagcaggagactctggttggccagaggggaagaaagctctggagaggcagccgctttgctgcccacaccacctagtgtgaagacagtccagagtcttgctactcctgatgcaagtccataaagcagtcctcccccatccgactgctgagggaaaacatgggcccctggaggaggtggcttttcttgtctgataaagttatataataaggtcttcacaagtttgctggtgtatggaagacatggacctcgcatcaaatacttgtggctgatgctctgtcgcaaaacttctttgtggaagagttggcaggaaaggaaaacaaccattgttgatatagcttctactgatatttcatatgtaatatctaagagtggaatatcagtgatcaactgcatcaaacagcacagcaattcttccaaaagatcttctgagtcagaactgtaattgccaggagatttttcttcataagtaaaatgaagttgtaattcctcctctgacatctgacagatgaacactttcagcaaacagcaaataataaacaaagcattgtgtgtctgccaaatgaagatgtggttctgacattctgctgaaagttttagttctttggttctagaaaggaagaccttaattagtgcaccaagatttcctgttcgaggattgttttcaactaatgacctgcagactgaaatggttgcttcctccaagagtttcaactcactactgctagttggtgcagggaaagaaaatgagagaagctgattccagaacgggtcattctcagagatagattccgtgcctgataactttttcaagtactcatttttaggaagatcgccgattctgctgctattcgatcccatcttctagcttaagcagataatttgtccttaaacctgcatttccaaaagacaacctgtctcagccggctgggggatctgctccagctccacggacccgcggacggatgggagggtggcagaggggtcaggagaagtcgctgtcgccgccgcagcccaggtggcgcacaccggctcaggcctccatgtttccacgtctcagcgggtacagatccggctccggtccggcctgcagctcggccccggctcggctccagcccgggccgcgtcggtgcggaggccaggaggcggcgagagaagaggg

SEQ ID NO: 9124 - RNA, 5927 nt, Homo sapiens
  source 1..5927: mol_type = other RNA
actggacttggagtcagaaggcctaataatcagtccctaaaatcaagtggcaactactgatattgcaggatagtgcctaggaaagaattaagagacccaaagggttgaccttgcagagactccagcctatgaagtatcagcaagtgccaaaaatttatggctctgcaaaaaagcacagggtgactcaattatgcagagagctctaccacccaatgcaaaaccctggctcccggaatctaaaggacgaaatgttgcttaaagtatgatatattaacaattccagtgcttaaaagtttccctcactaaatatttctcttggatgtaccttagcaagctcttaggaagttgctgagtgttctgatgctggtcctgtgtcctttccactttctatcgtctacttcccagctcctgtgctttccttccagagagaactgtgtgtgcagtgtactttctatgcttcaccttcagggaccttctcttctttcctttctctgtctttgtccttgagctgtgttgtctgcactgctgaatggtggcagtcctgctgcaaggttgttgttcatagattgtatgacaccagcctcaacgggtgactgtgggaactagagttagaaatctgaagctcttctgcaaagtgccttgaactcttgatagggaagatgctattgaaagggacaaattcttttaaaagtaaatattgtggcagaagtctttgttgataaaatgacacaatgcagtaacagcttcagatctggggtaaaatcagatgccaatttccatctgaacacacgatgatcctgtgttgcatcattacacatttttacttcgtgtaaaaatttctaagcaaactaatactcaaaattaatgcaagtataatgaaagtttatcattcagatttattgccatataataaatctttcacaaaaatcaggaagaagcctctggtgactttgcagagctgaggcagtgatgcacgtggtggggcctccctcctgagcgggaaccaggactgggagcatcacttgcaggcctccatggaggctgctgccccagctgagctgttagctagtgagtgcttctactgtgtgatgaatgagaaaagggaaagaggggagggcaatcagggttctgggggcacctcagtgagcccagaggcctggaggagaggctgtatgattccccagtcaggccttccttgggagtgtgccctctgtcaagatgactgggtttttgaagggcctcatttcctcacacaacaagcactgacagtcctgcagcccagggactgtcctgtggcactgcccagccctcagactcagaggacagttctgtggtcctgccagaagctcagctgttccacatgacccttaaacatttaaacaattttttggtttaaaggaaaaggaagccaatcaaaatgctttggaaacaaattaaagttgcaaattatttccccacatagtaaatacatatccttgctacctgaaatgataatcatcactccccctgctggctgagagcgcttctcctccttcagactggctctgccacaaagctaagtattagtagaagttgttgccaagcctcacctctagcctgtacatgggctctgaggtgaacacaggagtcagagtccccactccagcagtgactggaggaggcctgacagaacaagccccttggggacaggaggcaagctgcactcacctctgggaccccacccgggatgggcgctccacgagtcccttggccttagggaacctctgtttcattccatccagacgaggatagggaagcttcctgccctacctcgacagcctctaagagcacagcttggccaggccttcccgtgtggagcccacacagtggtgcactgagaggctgccagtgttttgaccttttacagagcttggggtgactgagaatggttcctccgaggccctcggaagatttgatggactcaaataacacgggcctgcagccctgggacacaggacaggagaagccagccctgacacagatgagctggcagtggattcgaacagtgtgctcagtctcgtctgggcttttgtgctttctatgttgaagaccaaatactttttctttgagaatgaaactaggctccttatctagactgtgaaggggcccgtgaggacacagagtgtgactggaaaggaaggtcccaactggccctcaatgtggccccagtggctgtttccctgcaagaagctccttcctccagctcaggcaccaacacacggatcacaccggcccagaaacaaagagcaaaacatgcttttcatcccacgtggaatacagtatgaacaaattactctcctttttctattagtgtgggtgaaggaaaaagactgttttcaaatgaagcttttctttttcccaatgattaatacagagtagattaacttaatttgtgctagactccaatttaattccagcaacagttcacaggccatattcacagaaaagttaatctgggcttcatgagaagtagccattttctttttcttttctttctttttttttttttgcgagacagggtctcactttgtggctcaggctggagtgtactggcacgttcttagctcactgcagccttgaactcctgggctcaggcaatcctcctaccttagcctcctgagtagctaggactacaggaatgtgccatcatgcctggctaatttttaagttttttgtagagatgggatctcactatgttgcccaagctggtttcagattcctgtgctcaagggattctgctaacttggctccccaaagtgctgggattacaaatgtgagccactgtatctggcccatattcttttttaagaaaagatgcagaggtgttaaatattaatatcaaattgtccaggcatggtgtttatgaaattgtgtgccctctgacaggcaaccaaacacacacgacttcatttctttattaattcctgcctcatcatcttttctcattgatgctccttaatgtcaaaggaatctctctctctcacacacacataagaccaaaacaaatatcttgaacatgcaaaaaaatagtctacgcttttgaatagtgtgcactgttgaatagtgtgcactgttggatagtgtgcactgttgaagtgtgatgtgcctaaggcaacaggatcttgggaaagctctagatttttggcttcgaaataaaactgcatgttgaatagcaggtttttacatttattattgttgtgtatttcctcccctttttgcaatactatctacgctgagttatctattgccaactagcaccaattctccaaatcaaagtgtgtgaggaaaacacactcgtgcaatcctctttaacagaagatacaccaagtaacctgtctgtctacttctgttacccagaaataaaagaacttgaagggctgcttggctggaggggtccgggtgggagagcatcctgccctcagtcggaatccatggtgaacagctggatgtcctgtggattccagtacaggccgactgctgagttgtagacaagagaccagacataggggataaaaaactcctcgggctgctcctcttccacatatttgaatttcaattctggaaatttcttcagtctgtctttgggcagcgcaacgacgccttgcttaatgatttccaggacccgttccactgacagctcagctccagcttgcagcaaccttgagctaaagaaggagatcaccagatcaatattttgcattatatcctgaaatgaaggatgagttcgaaattgttcaaagagatcgcgtttgtaaagcagggcgtataccaagtttgggttgtggtgaagggaatttgtcaggcaggagttgatgatctctaacatcattcgaatcacttcttcaatgacatttaggtcttgtgcataatctggtagaggaacatcattagaactcagcgaacctctcaaggactgtgtggcttgttccagaactttgttgtgttttttagacagcaaagaaaataaactggaagcataggatctgagaatgtgagagcaagttaaagacaagagttcctctccattgtcactgagggtcgagaagcaatgctgaagcgtagaacagtgagagtgggggaaatacagtttgtccaacacataaacatatctccgcaagtggcggcaggtataactgatgatcctctgggcagcatactgatggagagaacgaaactgtgccgacatatttgctaaagctgccaaacaatttgtgtgaaggtacttgtctcgtgtcctagtcatgttgtattgaatggttcttattaccaccaggatcaggagactccccaaggagatttcagttaaaactcgttctgaataccaagtaatattttttagtatcacttcatgaatggatctgttgaagccatcatcttccgtaaggatcaacaatattataagggccatatacacatggtgtgaattcctttcttcaacatgatacagaatctcaagaattggtaaaacaagattttccatatctgtgcgagccaacatgtatgttctaatattactattttgatggagcaaggtatacaagaggagagttgcttgatcagatgtctgctgttcacaaagagctgtgtacaaactattaaagttgatctggaaggcatgtggaattgatgaggggaaaggactgctatcttgtgtgttcttgaaggacataatggcttgtctgtaggggtttggcgcatctgaggcatctgtcagattggccaacaccagcagaagcaggagactctggttggccagaggggaagaaagctctggagaggcagccgctttgctgcccacaccacctagtgtgaagacagtccagagtcttgctactcctgatgcaagtccataaagcagtcctcccccatccgactgctgagggaaaacatgggcccctggaggaggtggcttttcttgtctgataaagttatataataaggtcttcacaagtttgctggtgtatggaagacatggacctcgcatcaaatacttgtggctgatgctctgtcgcaaaacttctttgtggaagagttggcaggaaaggaaaacaaccattgttgatatagcttctactgatatttcatatgtaatatctaagagtggaatatcagtgatcaactgcatcaaacagcacagcaattcttccaaaagatcttctgagtcagaactgtaattgccaggagatttttcttcataagtaaaatgaagttgtaattcctcctctgacatctgacagatgaacactttcagcaaacagcaaataataaacaaagcattgtgtgtctgccaaatgaagatgtggttctgacattctgctgaaagttttagttctttggttctagaaaggaagaccttaattagtgcaccaagatttcctgttcgaggattgttttcaactaatgacctgcagactgaaatggttgcttcctccaagagtttcaactcactgctagttggtgcagggaaagaaaatgagagaagctgattccagaacgggtcattctcagagatagattccgtgcctgataactttttcaagtactcatttttaggaagatcgccgattctgctgctattcgatcccatcttctagcttaagcagataatttgtccttaaacctgcatttccaaaagacaacctgtctcagccggctgggggatctgctccagctccacggacccgcggacggatgggagggtggcagaggggtcaggagaagtcgctgtcgccgccgcagcccaggtggcgcacaccggctcaggcctccatgtttccacgtctcagcgggtacagatccggctccggtccggcctgcagctcggccccggctcggctccagcccgggccgcgtcggtgcggaggccaggaggcggcgagagaagaggg

SEQ ID NO: 9125 - RNA, 1131 nt, Homo sapiens
  source 1..1131: mol_type = other RNA
actggacttggagtcagaaggccttggttcagaatcaactcctcctctttgagtttctgtttcttcctcagtaaaattaggcttcatttatcatgcaataaacatgtattgagtatgattgtgttcaggccctgtggctgggtgctagaggcccaaacacctgtactgcttctctcagagtggtaatgagaggatcaattcctaaatgcataaaaatataacaggaaatggaattccaggcactgagctgtgctttctgcagtttcattaagtagaggaaatgaaactggattcattgcaaagcaagtggtataatacggtggctaagaactcacgctcagtagccaaattgcctaagttgaaatcctggctccaccagaatttgggggatgttgctgaacctctcttcaattcagtttcctctgcctgtaaaatgggagtaagaactgtagatctcctcatgtggttgttgtgaggatttaatgagttattatgtgtaaaacacttaaagcagagtctagcacatagtgctcaatatacattagctattattgttattattatttgggacgtacaacacatcagaccacatgtttctaacacagacatgaccaagttgatatcagagagtgatctggttgtgataattttctctctattcgtggccaagcttcattcctgtcatctggccaatgaagtcaatgtccactcacttacttgctggtccatgaacatcctcctaaggctttctaactagaggagggagcctcagaaacaactactagaaactccagaccagccctccaggtccatgtggagaagaagatggggtagtcagctccctactaggaactactgattctgtccattatttcaagaggtataatgtgtttatcttattgctccaatcatgcatagcttcattcccaaaatctttacatggtctgtgatggctgtcagatttccagtcattctatttacgtttaaaattttttctaagtgatttatgcaatctgggtaaattaaggaaatggtccttatattgagcatttgtgtttagccaatattttgtatttttaaaacattttttgagatggagtcttgctctgttgcccaggctggagtgcaatg

SEQ ID NO: 9126 - RNA, 859 nt, Homo sapiens
  source 1..859: mol_type = other RNA
actggcagaacactgaagcagcaaagatgaccacctggttgagccaggtgtcagcacaggccaacttgaggacagacaggatttcacagaagaagtggttgatttcatggggcccacagaagggcagcctcaggatgagaaccacatggaccagggccagaagggaaccacatgcccaagaagtgacagccaggactgtgcacactccccatctcatgatgacagaatattgcagagggtggcagatagccatgtaccgatcgtaggacatcattaccaagatgagacactcagtgtgagcaaaagccatgtataaaaaggtctgcattgtgcatgggacaaaggagattgtttttctcttgttcaagccaaggtttgtcagcatcttggggacattgttggaagcatacgaaatatcaatgatggccaggtgtgagagaaagaagtacatgggggtgtgcagtctggagtccagccagatgagccccaggatggccccatttcccagcagggtgaagacgtataacagggagaaaagcccagagaggagcatctgaatccttaggctgagtggaaatcccaggagaatgaattctgtgacccatgtctgattttttgtcatgcccttgtgacagtacctgcgttggactctgctgtggcaatgagctatgtgtgtggtatcaggcctggtcttgtctcagaaatataattctatttagagaaattgtgcagagatcacaggagcttttgaaggccagagctgaggatcttgctcccaccagcagcccctgagagaaggaatttccagatgcaggagttgtctctcttttcttagcataggctgatgcagactgcagcc

SEQ ID NO: 9127 - RNA, 63 nt, Homo sapiens
  source 1..63: mol_type = other RNA
actggcattagtgggacttttaacattaaaaaaaaaaaaaaaaaaagtcccactaatgccagt

SEQ ID NO: 9128 - RNA, 540 nt, Homo sapiens
  source 1..540: mol_type = other RNA
actggcattagtgggactttttcatatctcttcactctgacaatttgatctctcattggcttgatatcctcagtgagtatacaaagctgaatccaaaatgaaatcacacctgaaaagactgttgattaaccaggctataaaccaggatgaaaccttggccgtttttgatgtagagatctctcatggaggcaaactgctcagttcctgcggtgtccagaatttccagcacggagggggaagagtccacttcgatctctttgcggtagaaatcttcaccaactcctaccagagggggggaaagatcaccccgctagctgtggcgcggctagacgaggcggaaggtgggcggaaatctgcgaactcttcggggcgagccgggtggcgctggagccgcgccctgctgagcgagcgagccggccggggacggtttcgggtcgggactccggcttcgggaacgggcctagtcttcaaaggagagtttagttcaatttctccttgacctcaggccggtgccatctctccagcgaagtccccagctct

SEQ ID NO: 9129 - RNA, 495 nt, Homo sapiens
  source 1..495: mol_type = other RNA
actggcattagtgggactttttcatatctcttcactctgacaatttgatctctcattggcttgatatcctgaaaagactgttgattaaccaggctataaaccaggatgaaaccttggccgtttttgatgtagagatctctcatggaggcaaactgctcagttcctgcggtgtccagaatttccagcacggagggggaagagtccacttcgatctctttgcggtagaaatcttcaatggtggggtcatatttctcaatgaaagtcccagtgacaaactgcacagtaagggcagatttgccaacccctccactccctaacaccactaccttgtattccctcatgagtctcaccttcaccaactcctaccagagggggggaaagatcaccccgctagctgtggcgcggctagacgaggcggaaggtgggcggaaatctgcgaactggggaggagagtgcagaggagcagagggcccaaccggggaagaagaggaagtt

SEQ ID NO: 9130 - RNA, 1265 nt, Homo sapiens
  source 1..1265: mol_type = other RNA
actggcattagtgggactttttcatatctcttcactctgacaatttgatctctcattggcttgatatcctgaaaagactgttgattaaccaggctataaaccaggatgaaaccttggccgtttttgatgtagagatctctcatggaggcaaactgctcagttcctgcggtgtccagaatttccagcacggagggggaagagtccacttcgatctctttgcggtagaaatcttcaatggtggggtcatatttctcaatgaaagtcccagtgacaaactgcacagtaagggcagatttgccaacccctccactccctaacaccactaccttgtattccctcatgagtctcaccttcaccaactcctaccagagggggggaaagatcaccccgctagctgtggcgcggctagacgaggcggaaggtgggcggaaatctgcgaactggggaggagagtgcagaggagcagagggcccaaccggggaagaagaggaagttacaggagggggaggggaaagagcgtagagtcggggagggtggggaagggatggtaatgcccttcctataggaactgcagcccgagcagggggcgtggggaggagggcgagcctgggaaaagcccggcgagggtggcgaggaggcgcgtgcccccgggagggaaagggtgggggctgcggcgaggggaccctgcggcgaggcggacgtcggaggagcccgcagcccggggctgcccggcactcctcccccgcccttcacacaaaggggcccagggaccccgcttcctgctcgcgcagcccagccggctcaggcctgagggctccgttccagttaccgctgcccgggcgggtttctgggccccggctcccgcgggggtcgtccggccccgccgtccgcacccgcccggccgccggggaggctctgtcacgccaaggccatggccacccgctggctcctctgtctctccgctgccccagcgctgccggaagggtttccctgacacactggctgaggtgccccagttccccgagactggacgggatcacttccggtggggaaagtcccacctcttcggggcgagccgggtggcgctggagccgcgccctgctgagcgagcgagccggccggggacggtttcgggtcgggactccggcttcgggaacgggcctagtcttcaaaggagagtttagttcaatttctccttgacctcaggccggtgccatctctccagcgaagtccccagctctggctccagctggcctgggccctgt

SEQ ID NO: 9131 - RNA, 1164 nt, Homo sapiens
  source 1..1164: mol_type = other RNA
actggcattagtgggactttttcatatctcttcactctgacaatttgatctctcattggcttgatatcctgaaaagactgttgattaaccaggctataaaccaggatgaaaccttggccgtttttgatgtagagatctctcatggaggcaaactgctcagttcctgcggtgtccagaatttccagcacggagggggaagagtccacttcgatctctttgcggtagaaatcttcaatggtggggtcatatttctcaatgaaagtcccagtgacaaactgcacagtaagggcagatttgccaacccctccactccctaacaccactaccttgtattccctcatgagtctcaccttcaccaactcctaccagagggggggaaagatcaccccgctagctgtggcgcggctagacgaggcggaaggtgggcggaaatctgcgaactggggaggagagtgcagaggagcagagggcccaaccggggaagaagaggaagttacaggagggggaggggaaagagcgtagagtcggggagggtggggaagggatggtaatgcccttcctataggaactgcagcccgagcagggggcgtggggaggagggcgagcctgggaaaagcccggcgagggtggcgaggaggcgcgtgcccccgggagggaaagggtgggggctgcggcgaggggaccctgcggcgaggcggacgtcggaggagcccgcagcccggggctgcccggcactcctcccccgcccttcacacaaaggggcccagggaccccgcttcctgctcgcgcagcccagccggctcaggcctgagggctccgttccagttaccgctgcccgggcgggtttctgggccccggctcccgcgggggtcgtccggccccgccgtccgcacccgcccggccgccggggaggctctgtcacgccaaggccatggccacccgctggctcctctgtctctccgctgccccagcgctgctcttcggggcgagccgggtggcgctggagccgcgccctgctgagcgagcgagccggccggggacggtttcgggtcgggactccggcttcgggaacgggcctctggaaacagtcttcaaaggagagtttagttcaatttctccttgacctcaggccggtgccatctctccagcgaagtccccagctct

SEQ ID NO: 9132 - RNA, 997 nt, Homo sapiens
  source 1..997: mol_type = other RNA
actggcattagtgggactttttcatatctcttcactctgacaatttgatctctcattggcttgatatcctgaaaagactgttgattaaccaggctataaaccaggatgaaaccttggccgtttttgatgtagagatctctcatggaggcaaactgctcagttcctgcggtgtccagaatttccagcacggagggggaagagtccacttcgatctctttgcggtagaaatcttcaatggtggggtcatatttctcaatgaaagtcccagtgacaaactgcacagtaagggcagatttgccaacccctccactccctaacaccactaccttgtattccctcatgagtctcaccttcaccaactcctaccagagggggggaaagatcaccccgctagctgtggcgcggctagacgaggcggaaggtgggcggaaatctgcgaactggggaggagagtgcagaggagcagagggcccaaccggggaagaagaggaagttacaggagggggaggggaaagagcgtagagtcggggagggtggggaagggatggtaatgcccttcctataggaactgcagcccgagcagggggcgtggggaggagggcgagcctgggaaaagcccggcgagggtggcgaggaggcgcgtgcccccgggagggaaagggtgggggctgcggcgaggggaccctgcggcgaggcggacgtcggaggagcccgcagcccggggctgcccggcactcctcccccgcccttcacacaaaggggcccagggaccccgcttcctgctcgcgcagcccagccggctcaggcctgagggctccgttccagttaccgctgcccgggcgggtttctgggccccggctcccgcgggggtcgtccggccccgccgtccgcacccgcccggccgccggggaggctctgtcacgccaaggccatggccacccgctggctcctctgtctctccgctgccccagcgctgctgctcgccgcggggaaagaa

SEQ ID NO: 9133 - RNA, 499 nt, Homo sapiens
  source 1..499: mol_type = other RNA
actggcattagtgggactttttcatatctcttcactctgacaatttgatctctcattggcttgatatcctgaaaagactgttgattaaccaggctataaaccaggatgaaaccttggccgtttttgatgtagagatctctcatggaggcaaactgctcagttcctgcggtgtccagaatttccagcacggagggggaagagtccacttcgatctctttgcggtagaaatcttcaccaactcctaccagagggggggaaagatcaccccgctagctgtggcgcggctagacgaggcggaaggtgggcggaaatctgcgaactcttcggggcgagccgggtggcgctggagccgcgccctgctgagcgagcgagccggccggggacggtttcgggtcgggactccggcttcgggaacgggcctagtcttcaaaggagagtttagttcaatttctccttgacctcaggccggtgccatctctccagcgaagtccccagctct

SEQ ID NO: 9134 - RNA, 855 nt, Homo sapiens
  source 1..855: mol_type = other RNA
actggcattagtgggactttttcatatctcttcactctgacaatttgatctctcattggcttgatatcctgaaaagactgttgattaaccaggctataaaccaggatgaaaccttggccgtttttgatgtagagatctctcatggaggcaaactgctcagttcctgcggtgtccagaatttccagcacggagggggaagagtccacttcgatctctttgcggtagaaatcttcaccaactcctaccagagggggggaaagatcaccccgctagctgtggcgcggctagacgaggcggaaggtgggcggaaatctgcgaactggggaggagagtgcagaggagcagagggcccaaccggggaagaagaggaagttacaggagggggaggggaaagagcgtagagtcggggagggtggggaagggatggtaatgcccttcctataggaactgcagcccgagcagggggcgtggggaggagggcgagcctgggaaaagcccggcgagggtggcgaggaggcgcgtgcccccgggagggaaagggtgggggctgcggcgaggggaccctgcggcgaggcggacgtcggaggagcccgcagcccggggctgcccggcactcctcccccgcccttcacacaaaggggcccagggaccccgcttcctgctcgcgcagcccagccggctcaggcctgagggctccgttccagttaccgctgcccgggcgggtttctgggccccggctcccgcgggggtcgtccggccccgccgtccgcacccgcccggccgccggggaggctctgtcacgccaaggccatggccacccgctggctcctctgtctctccgctgccccagcgctg

SEQ ID NO: 9135 - RNA, 5598 nt, Homo sapiens
  source 1..5598: mol_type = other RNA
actgggaagaggagctgagggaatggcttccagattgtggaccctggaccatggcaagagggcaagggatccaaggatgcacatggcaccaagcattctctgatggtgtagataaaagtaccactaggctaataaggtctgtgaacatttgtgtactcctactcaaagagggccataagaagaagagttgctctccacggcaaatatccagagtaaatggatttgaggccaaccccaccgctgttacagagcttgagaaatctttccatcaaagactctatctttattgaaaacacattcaacacttacccacaggcacgagccaggcggctgcctctgcatctgagggagcacacgtgtctggagcacctgcctgatgcaggctgaacacatacaactgcccccatttacaccacttggtcccatgagtaagttattactctgattttcaaatgaacttgactagtattcatttaagctccagaaagcatctggtgtcagaagaaaacaggaaggcaggatggttcactatttcccatttattcagcagcagtagttacactatcctcaatttgccctattttatgacaacctaacatattatgctgggaggaacagaatgagtatacaacaaggtttgccccagaagctaaaacaaatttactgacatttaaagagcaatactcaccctcggtttgtctacaggggaaagaaattcatccagtgatgcttcagtatgcaagaacaaaattgttttgcaataatacataagaaagaacattctctaggacaaaagtcccctccttgccaagagcctggggtgcagcaggagtacagtactttttttgaaaccctgaaggacagctcaattttttgctaagggcatgaaggttctggaatcagccatgtgtggagggatggatatgcctttttaaaaaagcatgacagtatttctgagcatgattttcagttgctaaatataggcttagcaacagcactgctgatgaaatcactcaggagacatttttaaagagaagcaaaagaaaacagatttgtgatgtacacacagcaggacaactgttttggatgaactcattccaacttgttaagacgacaaaaatgaccaacttgttaagatgagaaaaatgaacgtgttcaattaactgaatcctctttttaagacgactgagtgtgttgcagctgagtgaatctttgggactcgggaaaaataatccacacagacattgcaaatccctgtgttagcccaggcccaaactcctcacccaaatccaaagcctttcccgagggcagattttaccaggaacattcaccggggctggtaacctctcccatttctgtgtcagatgttcatagctgagtaacagataagcaaggaaaaagagcagggtccgagctaatctttatccacacatacgcccagagggccagtggctcatgtgggatgtgggtaccaagcttgagggctcagggtcacttctggaaacaaagctgacaggctgatggttcttactgacctgtcatagcttcctcagcagtctttcatcctaactgaaatatgacccactatggcaggggttcacgcccttggctgcaccctggaccttcttggggagctatagagaaatcctgatagcaggcctaccctggagattctgaggtaggcaagggtgagagacctgggcactaggaattttccaagctatgtaaatgattcttgtgtgcacatgtggtttagaaccacctcatcatgtcagccccactctggctttagggaactcaactcatcacctgacacaggctaacaaaggatcactgggtgcagtgggcccagaccaacagaattgggatcccctgggagagttgagaatgacttcaagagctattttagagacgcaacagagtgggtttgaggaataaggatgacagaggagttgaatgatgatgtaaaggttttccggcttggctagttaggtgattgtgacctcccaaccaagacagggagtataagagaatgagaaggtttgagagaaaagattagaattattttgaccattctggggttgagatttctgtgggtggtgacatatgatagcaagtttactgggccaaggccccatccagaggcagtcacagacctgagggctcttaagtatagaaggggcactagaggcatgggtctggacaagctcacctgggaaccaaggcagaggcaggatgagaagaagaaaatatgggaaatgatagcatttaaggaatggctagaagaagataattcagcaaatgacacacaaaaaaaaatggccagagaagttagaacagaaacagatggctgtggtgtaatgcaagctctgagaggacagggccatatctcggcttacttcgtatcctcggttcctggcccagggcctaccatgctgataaaatgtgagctcagcatcaataaaaatgtgctgagtcccagtttatgagtttacagaaggaaatggcggtcaactgtagctaaagctacagagtggtaaggtaaaaatgggaatgtttggtggctgagaggtctctggtgatggtgagagcagttgcagggaagagtgttgcttaataagccatgtatgacagttaaagcaccccaccctgggcatggttggggtacatgggggtgtgtgcacgtgtgggcaagagcacatgcgtatgtatgtgaatgcattcatggggcactactggagggccatggtatccaagtggctgctgggttgttcttgtttcctcctcagaactgtttcgcacttgggtatttttaaaaattcactcacatctgtgttccaccaattcagtaactgcagcacataaaaatgaagtaaaagatgcggagctagggcaaaacttttcatagcaaatgatgattttcaaaggtacaaatgcatggtccttagggttgcatgggacacaggattgcacatcagggatatgaaggtttggaatgaaagaaagcaaaagatgttgtggccaacatttccaactgctggttgctccagcacccgtgcctaggcagtgaggtggcccgccactggaaggtgcagtcacatgtccatgcccccaggcactgctccttcatcctctcttgcatccccaccctccttgggcttccagaccagatgggtgcccccagagcacctggctttacctgatgaggaggagcctgtccttttcagatggatggtcatccagccactgagagaagcgtgtgtgggaccactctgccctctggaaaggagatttcagttcagcgggtgctctcgtgaacaaaaactgaataatgatgctgaacggaatcacatcccccaatgcaggactactggctacatgttcacttgcctggaagagcagaggtctgaatgatctcagcatccgataggactttcctaaatcagatactcgtctacagaatggacccacagccaactccatctgtgcaaaatcagcagcaagtcgcattttcccaccttcaccaagaggtcttatgagactggcatggcggataaaaagttcaacagctctttgggcaatagcctcagtgttgtcaaagacaaaatccaagcattcaaagtgtttaaaatagtcactcataactctggcaatgaaaccttgtagctccttcatgtacagagaacaaggaacatcaggttttcctgagctggataatgacccagaaaagtcttcttgatgcatggtgatgattatggcctctatagcatctcccacagaagtgagtaagggttgcacagcattttccataagagcatgaatagcctttagagctgaaattatagtttgctcagctgccagtgggaatgagctctgactggaaacaacctttgttactgattggtgcaacttatacaatgaattcactactgccacatttcttctctgtccttcagtaagaggcccaatcacctgacttgcatctccttgtgtggagagaagctgctctgattttacactgtataactggatggtctttgccacattttttgacacagctaatgtgaggtttgtatcaacagcagcaacatttagttcacttgctatagttttaataataccatcaagttcatcagaggaaggaggattacgaccacccgggggaaaaaccaagttgataggatcgaagagtcgagataaggattttgatagataagcagcctcatagggttgtagtgagtctttcaaagccttttctggatcataatctggcttttttggtatgaatatatcttgtgcatcatcttccatgtgttgtaggtcaacatagaggtctgtagttccacttgcattaaaattcccttggatatgctgactgtattgttgaagacgcttccataagtcattataaagacgtaataatttagggtattctccttcaaatgcctgcttcaaaaacatcgaagagtttgttgccatatgaaattgagaagaaagtgcctgagtaactgaattccaaaatgtgtagaaaatttccggttgtccatccttaactatttcttcaatgaaacaaatgtgagaaacaggatctctcttcttggccaatactttttgtagatgttgtacctgtccacaaacagcataaatatgatccataagtttctccatattggtccagaatgaggcacgcaaagctgcagtatttcctggggttggcatggtagatcgtccaggtccccctctcacagctgactgggaaggctgagtcaaaacttttatgtctaatgcactgttgatattttcttctaaagtagcacaatatccatccacaacactggtaatagtatccttcaaagttccaagattatagaaaacctgaagagctgttccgacttgagttggattctgagtctccaaaccctgctctagtaggcgcttagcttgattttccacttcaagtcgggctcttgcaataaaaagtagatcattttctatcacttctattccagaaagatctattccttgagaaagataatcaagttcattgagactctgagcagcttttgttatctctctacttcccccttgcagttgtccttggagtctcttactgagattcaagatacgaataatcctccgaagcaaatcacaggcaacctgaagtcttgctagttgtgcagtccgggcaactatcttattgtatggttcaacaatttttgcttttatcctatcaacagctccctgtaaagccccaattctcgtctgcatcatctgaagaacaccttccaacgactcaatcccagttgcttgtgccagtaaatcttcatgtcttgcaacaacctgtaagtgtagttctctgtccaactgactgattccttgggcaagttttgctagttgttcagcaattacagcttgatgaatagattgagaagtataagtctttacatcaaagtcttcgtttaaaaagtcactataacacccgtcctgcagaagttcccggactgtagctgcagccgctccagagcctcgagctccgaggccagctacagcgacgctgccgccgccaccttccatgttggcaggtgccgggttgatgtc

SEQ ID NO: 9136 - RNA, 5886 nt, Homo sapiens
  source 1..5886: mol_type = other RNA
actgggcagggctgtggtgagtcggtgctggccgtgtgggcgaggtgacccgtcggtgacagggcctgctccctgcgaggtcgggtggtgcccgggccgggcggaggctcttctcgtgctcagggccggtttctggtgtgctcccgatgcgcttggctcttttctcgaggccgtgcttgtctgaggccaaccagggaccaggaggcagcgtcctggtgcccagcacctctcctcagtgtccctcgtccccacagaccggatcagggcctggcgagcctctgtgcctgccgtgcggtgtgaggacccgcggaccccaacccgcccttccctccgtcctgacccggcgccaggctcagctccagggcgaggtcctctggagtcatgttcgttctgcgtggcttggccgtgactgtggggactgggctgcccacggacagaaaggagaaacgcagcctgtgaccaggagacgcagcccagggtggagccgcgctggggccagggaggccgaggagggcaggagtccgagggtgtaagggtgccagggccttccgggtctcaggcttcgggacctggggagccaccctgtttggtgaccactcgtcctcggccttttcaacacaagggctttggagttgtgatgggctgttatcgggtgattccggtggccactcgtctgtgatcgggtgattccgatgactgctcgtctgtgatcgggcgattctggtgaccgctcgtctgtgatcgggtgagtccgatgactgctcgtctgtgatcgggtgattccgatgactgctcgtctgtgatcgggcgagtctggtgaccgctcgtctgtgatcgggtgagtccgatgactgctcgtctgtgatcgggtgattccgatgactgcttgtctgtgattgggcgattccggtggccgctcgtctgtgatcgggcgattccggtgaccgctcgtctgtgatcgggtgagtccgatgactgctcgtctgtgaccgggcgattccggtgaccgctcgtctgtgatcgggtgattccgaaccgcacattcagagttgttttcaaatgtttccgcacgttagttctgcctttcacacgcggtccagccaggttcagcgggggcacagggctgggcttgggcaccccccgccttccccaggccggtgaggtgacatcctaaaggagccacgaagcctgaggtccatttttccttgctctttatttccaggcactgaacttcccagccctgccgtggaagctgcctgccaggtcctccccatcctcaggtggaggcttctctgttgaggggcctcggagaccgccccccagccctcagcggaccatgctggctgggagctccgccctggggcttctgctctgctcaggtagggggagtccttccacggagctgtggccgcagcaggtgcactcttgggagtcggggaggcgggtggtgctcatgcgtgccagtgagggaggggcctcgccaccctcctgtactgtgagcctggccctgggcagccctctgccctggccagagcctgaccgtagccacgggctaacaggctctggaaaagtttccccaggactgccgcaggctcatccgcaggtagactccagaaccacggcccagcaggtcacacgtgtggctgtggctgtgtgcgtgccaagggacagtggcagtgtgccattgtgacagcgggtggccacacccgtcagcctccccaggagggagcaggagcgccggcttctccccaggtgcagacaggcaagggcgggccgcctgggtgtgtcctggcagtgtggagtgtcctggatgggctctgctcagccccctgctggcagagaaacccccacagacactgcaggactgggggtcctccctagtgtcctgctctccggcgggggggattggccaggagaggttaggctgagccattttgggagagttgaagaaggtgcttgggctgtggcaatgggaggtctgcgagcaaacagggtgcagctagtgaggacgggcgaacgggagggccgggcagaggctctgtcacgcggtgaggcgaggagtgtctcggcacttcgtgtctcttgcctggcaacaccacagggaccggacattctgaatcttcccagacccgctctgagaacataggcagccaccgcatcttctcaggaaagcaaagcgagcctactctaccctcacagtccaagccactgtggtcagccgggaagccgcccactgcccctgacggctttcgttttacctaggttgcccttggcacagagctggcctgtaggcatgtgtgcacaggtgtgtccatgtgaccggcttccccacacatgtgccaggcgcccagcacccccgccaggtggcctcactctgccctctgcccaggaaagcaggaaggccccgtggtgtccgctgcacacaggacaggcctcgggccccacagacacctcccacgtccggtgtggggccaattccgtgttagttgcctgctggttggggttagctcctgccaccctcagggctcctggaaggtgtctgccgctcaggaggtcagcacagcctcctgttgccatgacagccagctgctttaaaacgcccctttgacctgcaaaccacgtgcccagtgtggtgtgatccgcgagacactttggaaatggctgaggacgaggcaggtgtattaggagggtcagcgaactggggcccaaacctggtttgagaggggagtgctgggggcatccggtaggaggaggggcaggagggaggcctgggcctggccgccccccagccccctctggggcacccgtctgagttctgccccagttagtacaggaatgtaatgaagtgcgaggtgacagagtccctgctctggggacaccggcagtgccgcgaggcatggagcgggggctacttgcccccttgcaccttctggtcgtaggtgcctgcgtgcttgtagccggacacatagcctgactcgtccaccagatccacgcggccagccttgcccttgcccttgccagaggggtcgaagcgctccttgtgggagcccgtgaacttggtggtgtccgtgagcctcgacactgtgggcgacgagatggctttcgtcacccctgagatgatgggcgccttgccctcgatgagcctgtgcacctcgcgaacggcctcctcgctgctcttgtctttgaatcgcttcttggcgagctcctccagcgcctcctggaactgctcaaaggtgatggtccggcaagacttccctttgatcttgctgaagacgatgtccacgtcagtgacggtcacgttcctgccgtcgatcacctggcagtccttgcacagcttcgaccagttcttgccgtgcatctccctcccggtggccctggcgtccccgtgcacggcaaagcgccggaaggcctcctccagggcactgagctcaggggatgcggctgccccctcaccagcaccctccgattccagcgacagcctcttggctgcccggtccttcgaggggtcccccggggacttggggggcgtcctgttggcagctttggcaggcttggccttgtcagccatgttgccctttccctggaaggcaccaaaaatgcagatgccaacccagcggaggatgcaggggcaggatcctggtgggggctgggccgcgtgggggcaggatcctgggggtggaagggccgcctgggggcaggatcctgggggtggaagggccaggtcaggtgtcgagctgggaacagtttccagttttatcgctgacaccatttctttgtctgaaacaggagcttctcacaggcctggtctgtgtttcccctgggcctctgcagcaggggtcgctggacaggaggagcagctgagaaattaccagaagcaatggtgggttttgtgagcacccagaacagtggtgggtgtgcgggtcagagagaaagaaccttctgggatgcttcaaactcagggctgcgttctgtggtctcatctcctgtggggacgcgcctgaacagagacccttattcacacacctcagagagtcatctgagaacctgcaccccgtggggcccgcctgggagcaaagggatgagggaagcccctcagagccaccttcagggctcacgcaggacttcccagcccatcagcacgtgctttgcatgaggttttgataagcttggaggttggccttggagggctgagcgggacataaaacgtcctgccctcatgaggccttcagttgggacaagtgataaacaaataagcaatgacacatcaggcagcgaggagtgaagaggagaaactgaggcaggtcagagggaggccagcaggcgatttcagacctggcggaagagaatgtgcgtgagcagagatgcggacgggtgggagtcacgacgcgtgagaacggtccggcccgcggcccctgcgcccctgctgggcaggcaccacctgtgctaggctcagcccctctcagcacagcaagcagcatgagatggcacgcatgagagcacggtgggggccgtgggggagagggcagaaaggaacaggggtcaggccatcgccggatctactgaagacagacactgccttcaaacgttctgaggaaaaatgcttcaggctgggacttggatacccacgtccactgtcccactcaggctgaggggagcaaggccacctgcagtgggtgtgacctcagagacgtggccacaccccctgcggaggtgcttggtgactgggcttcccaggaagacgagggtgacagccgtcaacagccgagaagaagtagtagatgcaggaacccatggccgtcacacgggagtgagtccacgggcgcttgggagggctgagaaccaggcccaggcagttccggagggaaaagtggaacccgtcccaactcagccccagcctttctgcaccaaggggtggagcagtgccgacctcagacgccagctgccagaaatgcttccaaagcccgcctctgcgtggggtgtgtgctgaggggtctcacgtggggactcgcctcagagcccatctgagcttcactgttctaggttcttgtagttttgttttacctcaaacatgcattagcttaacaaaatattttttaaaaggtttttaaactaaaaatgacaatgaattaggcacgacgtgccgctgtgggaagtcagccaggctgctgctgggtctggaggagcaggacacgggccacagacacggagcaggagtggaggagatgggagccacactgtctggatcgcttcattagacccacgtgctgtttccacaatgacggtaataagaatacatttaattttgagagaacatggaggtgtcagacggacaacgagcctgggtgggcgcctctcccttggcgctctccaccgagcatggcatgctgctgtgccagctgcttctccttggatgggcagaggccaggtgtcctccactttcccagtttctgggcacagcacacctgagccctgggtgcagaccctcacaccatttcccccagaggctctgctctttcaccgtgagggaaaagaaggttgtgtagcagaagagactccaggaagacaaactgctcacctggggtcaaaggacaagctcccaggcgtgtacccaccatctccacgcgtgtgccctgagcccccagggggtcaccctgcactcccaggcctgtgcccaccatcccacatgtgcccagcactcccaggcctgtgcccgccatcccagttgtgcctgtactcccaggcctgtgtcttgcatccagatgtgcacctgcaccctctcccactggccggcacctccctggtaggagggacgtgccaagccctgacctgacccaggtgtctgctcacagcacatgccccttccctggccagaccctatgggaccac

SEQ ID NO: 9137 - RNA, 3755 nt, Homo sapiens
  source 1..3755: mol_type = other RNA
actgggcagggctgtggtgagtcggtgctggccgtgtgggcgaggtgacccgtcggtgacagggcctgctccctgcgaggtcgggtggtgcccgggccgggcggaggctcttctcgtgctcagggccggtttctggtgtgctcccgatgcgcttggctcttttctcgaggccgtgcttgtctgaggccaaccagggaccaggaggcagcgtcctggtgcccagcacctctcctcagtgtccctcgtccccacagaccggatcagggcctggcgagcctctgtgcctgccgtgcggtgtgaggacccgcggaccccaacccgcccttccctccgtcctgacccggcgccaggctcagctccagggcgaggtcctctggagtcatgttcgttctgcgtggcttggccgtgactgtggggactgggctgcccacggacagaaaggagaaacgcagcctgtgaccaggagacgcagcccagggtggagccgcgctggggccagggaggccgaggagggcaggagtccgagggtgtaagggtgccagggccttccgggtctcaggcttcgggacctggggagccaccctgtttggtgaccactcgtcctcggccttttcaacacaagggctttggagttgtgatgggctgttatcgggtgattccggtggccactcgtctgtgatcgggtgattccgatgactgctcgtctgtgatcgggcgattctggtgaccgctcgtctgtgatcgggtgagtccgatgactgctcgtctgtgatcgggtgattccgatgactgctcgtctgtgatcgggcgagtctggtgaccgctcgtctgtgatcgggtgagtccgatgactgctcgtctgtgatcgggtgattccgatgactgcttgtctgtgattgggcgattccggtggccgctcgtctgtgatcgggcgattccggtgaccgctcgtctgtgatcgggtgagtccgatgactgctcgtctgtgaccgggcgattccggtgaccgctcgtctgtgatcgggtgattccgaaccgcacattcagagttgttttcaaatgtttccgcacgttagttctgcctttcacacgcggtccagccaggttcagcgggggcacagggctgggcttgggcaccccccgccttccccaggccggtgaggtgacatcctaaaggagccacgaagcctgaggtccatttttccttgctctttatttccaggcactgaacttcccagccctgccgtggaagctgcctgccaggtcctccccatcctcaggtggaggcttctctgttgaggggcctcggagaccgccccccagccctcagcggaccatgctggctgggagctccgccctggggcttctgctctgctcaggtagggggagtccttccacggagctgtggccgcagcaggtgcactcttgggagtcggggaggcgggtggtgctcatgcgtgccagtgagggaggggcctcgccaccctcctgtactgtgagcctggccctgggcagccctctgccctggccagagcctgaccgtagccacgggctaacaggctctggaaaagtttccccaggactgccgcaggctcatccgcaggtagactccagaaccacggcccagcaggtcacacgtgtggctgtggctgtgtgcgtgccaagggacagtggcagtgtgccattgtgacagcgggtggccacacccgtcagcctccccaggagggagcaggagcgccggcttctccccaggtgcagacaggcaagggcgggccgcctgggtgtgtcctggcagtgtggagtgtcctggatgggctctgctcagccccctgctggcagagaaacccccacagacactgcaggactgggggtcctccctagtgtcctgctctccggcgggggggattggccaggagaggttaggctgagccattttgggagagttgaagaaggtgcttgggctgtggcaatgggaggtctgcgagcaaacagggtgcagctagtgaggacgggcgaacgggagggccgggcagaggctctgtcacgcggtgaggcgaggagtgtctcggcacttcgtgtctcttgcctggcaacaccacagggaccggacattctgaatcttcccagacccgctctgagaacataggcagccaccgcatcttctcaggaaagcaaagcgagcctactctaccctcacagtccaagccactgtggtcagccgggaagccgcccactgcccctgacggctttcgttttacctaggttgcccttggcacagagctggcctgtaggcatgtgtgcacaggtgtgtccatgtgaccggcttccccacacatgtgccaggcgcccagcacccccgccaggtggcctcactctgccctctgcccaggaaagcaggaaggccccgtggtgtccgctgcacacaggacaggcctcgggccccacagacacctcccacgtccggtgtggggccaattccgtgttagttgcctgctggttggggttagctcctgccaccctcagggctcctggaaggtgtctgccgctcaggaggtcagcacagcctcctgttgccatgacagccagctgctttaaaacgcccctttgacctgcaaaccacgtgcccagtgtggtgtgatccgcgagacactttggaaatggctgaggacgaggcaggtgtattaggagggtcagcgaactggggcccaaacctggtttgagaggggagtgctgggggcatccggtaggaggaggggcaggagggaggcctgggcctggccgccccccagccccctctggggcacccgtctgagttctgccccagttagtacaggaatgtaatgaagtgcgaggtgacagagtccctgctctggggacaccggcagtgccgcgaggcatggagcgggggctacttgcccccttgcaccttctggtcgtaggtgcctgcgtgcttgtagccggacacatagcctgactcgtccaccagatccacgcggccagccttgcccttgcccttgccagaggggtcgaagcgctccttgtgggagcccgtgaacttggtggtgtccgtgagcctcgacactgtgggcgacgagatggctttcgtcacccctgagatgatgggcgccttgccctcgatgagcctgtgcacctcgcgaacggcctcctcgctgctcttgtctttgaatcgcttcttggcgagctcctccagcgcctcctggaactgctcaaaggtgatggtccggcaagacttccctttgatcttgctgaagacgatgtccacgtcagtgacggtcacgttcctgccgtcgatcacctggcagtccttgcacagcttcgaccagttcttgccgtgcatctccctcccggtggccctggcgtccccgtgcacggcaaagcgccggaaggcctcctccagggcactgagctcaggggatgcggctgccccctcaccagcaccctccgattccagcgacagcctcttggctgcccggtccttcgaggggtcccccggggacttggggggcgtcctgttggcagctttggcaggcttggccttgtcagccatgttgctccctcggctccgtttacgtaaccgaaaccgcagaataaagggctcctcagatcttcgggcgctgctcccaggggtgcgggaaggtgtcccggcagcgcctctccatcgccacaggcccgcggacagtagccaagacccggggcagctggaggctctgcggggggcggtctgacagccccac

SEQ ID NO: 9138 - RNA, 3655 nt, Homo sapiens
  source 1..3655: mol_type = other RNA
actgggcagggctgtggtgagtcggtgctggccgtgtgggcgaggtgacccgtcggtgacagggcctgctccctgcgaggtcgggtggtgcccgggccgggcggaggctcttctcgtgctcagggccggtttctggtgtgctcccgatgcgcttggctcttttctcgaggccgtgcttgtctgaggccaaccagggaccaggaggcagcgtcctggtgcccagcacctctcctcagtgtccctcgtccccacagaccggatcagggcctggcgagcctctgtgcctgccgtgcggtgtgaggacccgcggaccccaacccgcccttccctccgtcctgacccggcgccaggctcagctccagggcgaggtcctctggagtcatgttcgttctgcgtggcttggccgtgactgtggggactgggctgcccacggacagaaaggagaaacgcagcctgtgaccaggagacgcagcccagggtggagccgcgctggggccagggaggccgaggagggcaggagtccgagggtgtaagggtgccagggccttccgggtctcaggcttcgggacctggggagccaccctgtttggtgaccactcgtcctcggccttttcaacacaagggctttggagttgtgatgggctgttatcgggtgattccggtggccactcgtctgtgatcgggtgattccgatgactgctcgtctgtgatcgggcgattctggtgaccgctcgtctgtgatcgggtgagtccgatgactgctcgtctgtgatcgggtgattccgatgactgctcgtctgtgatcgggcgagtctggtgaccgctcgtctgtgatcgggtgagtccgatgactgctcgtctgtgatcgggtgattccgatgactgcttgtctgtgattgggcgattccggtggccgctcgtctgtgatcgggcgattccggtgaccgctcgtctgtgatcgggtgagtccgatgactgctcgtctgtgaccgggcgattccggtgaccgctcgtctgtgatcgggtgattccgaaccgcacattcagagttgttttcaaatgtttccgcacgttagttctgcctttcacacgcggtccagccaggttcagcgggggcacagggctgggcttgggcaccccccgccttccccaggccggtgaggtgacatcctaaaggagccacgaagcctgaggtccatttttccttgctctttatttccaggcactgaacttcccagccctgccgtggaagctgcctgccaggtcctccccatcctcaggtggaggcttctctgttgaggggcctcggagaccgccccccagccctcagcggaccatgctggctgggagctccgccctggggcttctgctctgctcaggtagggggagtccttccacggagctgtggccgcagcaggtgcactcttgggagtcggggaggcgggtggtgctcatgcgtgccagtgagggaggggcctcgccaccctcctgtactgtgagcctggccctgggcagccctctgccctggccagagcctgaccgtagccacgggctaacaggctctggaaaagtttccccaggactgccgcaggctcatccgcaggtagactccagaaccacggcccagcaggtcacacgtgtggctgtggctgtgtgcgtgccaagggacagtggcagtgtgccattgtgacagcgggtggccacacccgtcagcctccccaggagggagcaggagcgccggcttctccccaggtgcagacaggcaagggcgggccgcctgggtgtgtcctggcagtgtggagtgtcctggatgggctctgctcagccccctgctggcagagaaacccccacagacactgcaggactgggggtcctccctagtgtcctgctctccggcgggggggattggccaggagaggttaggctgagccattttgggagagttgaagaaggtgcttgggctgtggcaatgggaggtctgcgagcaaacagggtgcagctagtgaggacgggcgaacgggagggccgggcagaggctctgtcacgcggtgaggcgaggagtgtctcggcacttcgtgtctcttgcctggcaacaccacagggaccggacattctgaatcttcccagacccgctctgagaacataggcagccaccgcatcttctcaggaaagcaaagcgagcctactctaccctcacagtccaagccactgtggtcagccgggaagccgcccactgcccctgacggctttcgttttacctaggttgcccttggcacagagctggcctgtaggcatgtgtgcacaggtgtgtccatgtgaccggcttccccacacatgtgccaggcgcccagcacccccgccaggtggcctcactctgccctctgcccaggaaagcaggaaggccccgtggtgtccgctgcacacaggacaggcctcgggccccacagacacctcccacgtccggtgtggggccaattccgtgttagttgcctgctggttggggttagctcctgccaccctcagggctcctggaaggtgtctgccgctcaggaggtcagcacagcctcctgttgccatgacagccagctgctttaaaacgcccctttgacctgcaaaccacgtgcccagtgtggtgtgatccgcgagacactttggaaatggctgaggacgaggcaggtgtattaggagggtcagcgaactggggcccaaacctggtttgagaggggagtgctgggggcatccggtaggaggaggggcaggagggaggcctgggcctggccgccccccagccccctctggggcacccgtctgagttctgccccagttagtacaggaatgtaatgaagtgcgaggtgacagagtccctgctctggggacaccggcagtgccgcgaggcatggagcgggggctacttgcccccttgcaccttctggtcgtaggtgcctgcgtgcttgtagccggacacatagcctgactcgtccaccagatccacgcggccagccttgcccttgcccttgccagaggggtcgaagcgctccttgtgggagcccgtgaacttggtggtgtccgtgagcctcgacactgtgggcgacgagatggctttcgtcacccctgagatgatgggcgccttgccctcgatgagcctgtgcacctcgcgaacggcctcctcgctgctcttgtctttgaatcgcttcttggcgagctcctccagcgcctcctggaactgctcaaaggtgatggtccggcaagacttccctttgatcttgctgaagacgatgtccacgtcagtgacggtcacgttcctgccgtcgatcacctggcagtccttgcacagcttcgaccagttcttgccgtgcatctccctcccggtggccctggcgtccccgtgcacggcaaagcgccggaaggcctcctccagggcactgagctcaggggatgcggctgccccctcaccagcaccctccgattccagcgacagcctcttggctgcccggtccttcgaggggtcccccggggacttggggggcgtcctgttggcagctttggcaggcttggccttgtcagccatgttgctgcatccctgaataaggtttacctaggtgtggatttcttctttttagttatgcagctcgtcataaatcaactcttcatatac

SEQ ID NO: 9139 - RNA, 3647 nt, Homo sapiens
  source 1..3647: mol_type = other RNA
actgggcagggctgtggtgagtcggtgctggccgtgtgggcgaggtgacccgtcggtgacagggcctgctccctgcgaggtcgggtggtgcccgggccgggcggaggctcttctcgtgctcagggccggtttctggtgtgctcccgatgcgcttggctcttttctcgaggccgtgcttgtctgaggccaaccagggaccaggaggcagcgtcctggtgcccagcacctctcctcagtgtccctcgtccccacagaccggatcagggcctggcgagcctctgtgcctgccgtgcggtgtgaggacccgcggaccccaacccgcccttccctccgtcctgacccggcgccaggctcagctccagggcgaggtcctctggagtcatgttcgttctgcgtggcttggccgtgactgtggggactgggctgcccacggacagaaaggagaaacgcagcctgtgaccaggagacgcagcccagggtggagccgcgctggggccagggaggccgaggagggcaggagtccgagggtgtaagggtgccagggccttccgggtctcaggcttcgggacctggggagccaccctgtttggtgaccactcgtcctcggccttttcaacacaagggctttggagttgtgatgggctgttatcgggtgattccggtggccactcgtctgtgatcgggtgattccgatgactgctcgtctgtgatcgggcgattctggtgaccgctcgtctgtgatcgggtgagtccgatgactgctcgtctgtgatcgggtgattccgatgactgctcgtctgtgatcgggcgagtctggtgaccgctcgtctgtgatcgggtgagtccgatgactgctcgtctgtgatcgggtgattccgatgactgcttgtctgtgattgggcgattccggtggccgctcgtctgtgatcgggcgattccggtgaccgctcgtctgtgatcgggtgagtccgatgactgctcgtctgtgaccgggcgattccggtgaccgctcgtctgtgatcgggtgattccgaaccgcacattcagagttgttttcaaatgtttccgcacgttagttctgcctttcacacgcggtccagccaggttcagcgggggcacagggctgggcttgggcaccccccgccttccccaggccggtgaggtgacatcctaaaggagccacgaagcctgaggtccatttttccttgctctttatttccaggcactgaacttcccagccctgccgtggaagctgcctgccaggtcctccccatcctcaggtggaggcttctctgttgaggggcctcggagaccgccccccagccctcagcggaccatgctggctgggagctccgccctggggcttctgctctgctcaggtagggggagtccttccacggagctgtggccgcagcaggtgcactcttgggagtcggggaggcgggtggtgctcatgcgtgccagtgagggaggggcctcgccaccctcctgtactgtgagcctggccctgggcagccctctgccctggccagagcctgaccgtagccacgggctaacaggctctggaaaagtttccccaggactgccgcaggctcatccgcaggtagactccagaaccacggcccagcaggtcacacgtgtggctgtggctgtgtgcgtgccaagggacagtggcagtgtgccattgtgacagcgggtggccacacccgtcagcctccccaggagggagcaggagcgccggcttctccccaggtgcagacaggcaagggcgggccgcctgggtgtgtcctggcagtgtggagtgtcctggatgggctctgctcagccccctgctggcagagaaacccccacagacactgcaggactgggggtcctccctagtgtcctgctctccggcgggggggattggccaggagaggttaggctgagccattttgggagagttgaagaaggtgcttgggctgtggcaatgggaggtctgcgagcaaacagggtgcagctagtgaggacgggcgaacgggagggccgggcagaggctctgtcacgcggtgaggcgaggagtgtctcggcacttcgtgtctcttgcctggcaacaccacagggaccggacattctgaatcttcccagacccgctctgagaacataggcagccaccgcatcttctcaggaaagcaaagcgagcctactctaccctcacagtccaagccactgtggtcagccgggaagccgcccactgcccctgacggctttcgttttacctaggttgcccttggcacagagctggcctgtaggcatgtgtgcacaggtgtgtccatgtgaccggcttccccacacatgtgccaggcgcccagcacccccgccaggtggcctcactctgccctctgcccaggaaagcaggaaggccccgtggtgtccgctgcacacaggacaggcctcgggccccacagacacctcccacgtccggtgtggggccaattccgtgttagttgcctgctggttggggttagctcctgccaccctcagggctcctggaaggtgtctgccgctcaggaggtcagcacagcctcctgttgccatgacagccagctgctttaaaacgcccctttgacctgcaaaccacgtgcccagtgtggtgtgatccgcgagacactttggaaatggctgaggacgaggcaggtgtattaggagggtcagcgaactggggcccaaacctggtttgagaggggagtgctgggggcatccggtaggaggaggggcaggagggaggcctgggcctggccgccccccagccccctctggggcacccgtctgagttctgccccagttagtacaggaatgtaatgaagtgcgaggtgacagagtccctgctctggggacaccggcagtgccgcgaggcatggagcgggggctacttgcccccttgcaccttctggtcgtaggtgcctgcgtgcttgtagccggacacatagcctgactcgtccaccagatccacgcggccagccttgcccttgcccttgccagaggggtcgaagcgctccttgtgggagcccgtgaacttggtggtgtccgtgagcctcgacactgtgggcgacgagatggctttcgtcacccctgagatgatgggcgccttgccctcgatgagcctgtgcacctcgcgaacggcctcctcgctgctcttgtctttgaatcgcttcttggcgagctcctccagcgcctcctggaactgctcaaaggtgatggtccggcaagacttccctttgatcttgctgaagacgatgtccacgtcagtgacggtcacgttcctgccgtcgatcacctggcagtccttgcacagcttcgaccagttcttgccgtgcatctccctcccggtggccctggcgtccccgtgcacggcaaagcgccggaaggcctcctccagggcactgagctcaggggatgcggctgccccctcaccagcaccctccgattccagcgacagcctcttggctgcccggtccttcgaggggtcccccggggacttggggggcgtcctgttggcagctttggcaggcttggccttgtcagccatgttgcttggagacgcagcgactgcagcggaggcgcctccgcgactcggccgcgcgcgacccggtgctcagcggagctct

SEQ ID NO: 9140 - RNA, 4683 nt, Homo sapiens
  source 1..4683: mol_type = other RNA
actgggcagggctgtggtgagtggggcagctggggtgagggctggcctgtgggtgggggtcctggggctttcctgtgacagctgtggctcctcatcactgggagtgggcaacccttgactgggagggagggtctcattgccaagggcctctgtgggaacccaaactgctggctccacacagtcctccaagtagacacatctctgtgtgacttcatccaggacctggggggtggggcacacagggacacagccttctaccctgggtacgtcccggcagctggctgcccgtgggtcccggcaggtttggaagcaggggctggcacaggcatcgtagcgccactcgcagatggggtaggcagcccccgagggcttggcatccagaaggcggaagagtgtgccccggcggaacacctctgtgtgttcgtacagccgcagggccagcaccgcgcccgacacatagaggaaggagctgggcttggccagggactccagggccaccaggcctgcctgccgtgtcccccggtgcagcaagaaggaggcatgctgttggaaggtgtcacggccctgccacttagccagctccagagacccgttggctgtgacgtgaaggaagaagttgggtctgtctgctgcctccagggacaccacatctgggtcatgggccttggccttgtacagagcagctgtcagcaggaagctcacaatgtctgctggcgccacatcctctgtcctcactaggactatgtcatcgcccaccgccttcatgcccaccagagcaccaccggctgccaagctggatagctgataggggcccttacctagcactttgttaaagaagtcacagtcatacgggcagaggcggggggttcgccagtcaacagccaccccatgctggcaacactggtgggcataagcggagacgctggcacagaagcactcacagtcaccaccctggctgcagccacatgtgtctgtcaggcagtttgagtaaaaccaagtgacatcaaccacagggtggcagatctcaaacacctcactgagcaggatgctgcactccttcttggcaaatggttctcggagaggattcaggacacacatatcccgaggatcgagggtgtctgggcactcaactgcagcccaactgctgccaaactcctgggggttagttagctctaggttctccggggtcctcatctcattgatggtttttaagtcaaagttcccacagaggcccgccagctggccctgccactgaggcccagcctggacgtgcactgtggttctctggtcccacaagagggtgatgtgctcctgtgggaaatgcaccagtgtgaaaaatcccactcgccatgtgtggacctcctgcttgtcatccaggaagctctctggactaggatttccggagtcatcatcaaagacaatgagtgagttcccaacgttgatggaaataaatttcctgcagatcatgccagagctgtagcagttcacattctctacaatcacagagaagctgacatctgatgtgctcttgaccaggtgcactttgcatgcccccacgaagtcaaacgggagcccatcaaacgtgcggtaatgccggtccccataggcagtgcaggtggaggcgcaagggtgcagggtgcactggaatgagccccgctggcacacacaggtatggcaaggagacatcacctggtccccagggaaatactccttccccttccaagtgcaggggcactcctctggcaggaaacatgcatccccgtgtctgagcagaccctggggacaggcgcagcccgagaggcaggggccacgggctgacacgctcaggttcagcagttgctgctcacacgtcctctccctgctcagctccaggtccgtgtgcaggtcgctgcagttcacgaagacctggcctgctgggcaggcagcagctggggctctgctatcacagctcatgactccatctttgcagtggcagtggcccagggatgggatgtcactgtctccggggggatagtccactccctggaagtggcaggagcactggttccgggggacacagaggtcagcctgggtgtccagataggtgtccggtgggcaggcacagccctccacacactcgtctctgctcaggtcatcgccaccatcaaccccacaggcctcagggctggccaggtcctggcaggtacgtccacacggggccacgcaggggctatactccttggaggcctcacaggacagtgcacaggctggcaggcgggcgcggaaatcaacggggagcccatggcgccggcacaggtgggcgtagtgggccagtgtggcgcacaggcagggctgcccgcagcggcaggcatccctgcggcactgctcaaagtagggcacggggctcaggaacgcagagcagggcgcaaacatctcccccgtgagcacgctgcaggcctgcactgagtaggaggcggcttgcaggtgcacatcgcaggggtccagaggggagccagagaccagcggggagcaagcagaaagtgttttccaggaattgccaaaaagttgtggggtgctctcaggtacacccactggagacaggaagtcatcctgcgtgttgccattgaaggtgccgcagaggcccacggtatcctccacccatcgctggtccacttgcaggtacagtcggagcccttcacggtcgtagagcacccgcacgcccacgttcgtcctcacccgcaggaacacggaggacagcctacggatctcaaaggcatcatctgtgtatggcgggatgatcttgtactggtcaaacagaaggacatcccctgcctgggtcagggtcacctgcctccgagggtcctggtgcagaatcactgacactgactggacacaggctccatcttggttcaggccacatggggcattctgcaatgtcacggtgaaggtgcccgaagagcggctcttggccaggatgtactgacatgtggcggggaacgtgtaccggcggccatcaaaggttgtgaagtgaatgtcaccagtcactgagcactcagctgggcagacagctgtgctgcactcccacttgcctgaggtgcatgtgcaagtattgcagtcttccttcaccacagagccaggtgggtacagagtcccgtgaaactcacagggacactcagctggtgccacgcagcccccatcctcgaagatgagcccattggggcaatagcagccgtccacacaggcgatctcactgtccacacaggatgcccggggatggcaggaggcagggcagcaggcgatgcactcattgtaggtaaaggccttctccttgcagtgcacagtgcattgccggagctgggtcctccagccttgcaagggccgccctgcctgggcacacgcccgggcatactccgccagtgcccggcaccaggtggctacatcacccattgattggcagagatcactggtacaactggctgtgaagggcagagggctgacgtaggcgtggcaggcgtcaaaggggggccgcagtagagcctcacactgctcgtacacgccctgcatggttcctgggttctgctgtaggcacggtgggcgaggcagggaggaagttgtgggccctggaggctggttaggggcctgctcctgccagctgtgcacaaactcaaccacgtcgtcagtcagcttcccagagctggtcaccagatcatccttggggtcagcattgttgttcccacacagcccatgggtccagcccagaagctctggactcatcttgatgtagacagccgaggcaccatcccaggccagtgtgaaggctgactgatgccgcacgatgacatagccggcaagctgctgcagacgcgcgctccccatgacatgtggcagttggaccctcatgcctccatgggtgacctccttggccagatggatctcctgctcacccacaaagaagaggctgacagccctggagcaggtgtagggtgaagagccacactgcgggtcattgtgtacctggatggagaagctctgtccctcgggctcatggcgacccaccagggtgtagctgccctttccggagaggtagtagtagagcccatcaaatgtctccacgtggtgctgcccccacgcccggcaaatgctgtccctctcagggccggcattgtacaccatctggcagcgcggtccagtggcattgaagcgtctgcagtcacagaaggctgggtgcacacactcgcctccattgaagcaggagaacaagtaggatggtgcacacttggcccgatggagccgcctttcccaggaagacatggccacggagtctggggcttcagcctgctggcctcccacgactgtagccttgtcccccatggcaagggtcgcctcctggtggctgctgctggaggaaacacgagtctgcgcgggcccattcctcattcctttaacgtttctcattcctcgagcccccgacctccctgagtccacaaccctctcaccgaggcgctgcacccgcagggactcggctgcctgctcaccccagggcagccagacacaaagcagccagcagagcgcagacgccaggactcccatagggacacgaggggaccggaggacttgagcgcagggccagcctcccgaggtgcctccccgggctaaggcagggtcacacctccactccgcagccgaggtccctcttgttctcat

SEQ ID NO: 9141 - RNA, 4647 nt, Homo sapiens
  source 1..4647: mol_type = other RNA
actgggcagggctgtggtgagtggggcagctggggtgagggctggcctgtgggtgggggtcctggggctttcctgtgacagctgtggctcctcatcactgggagtgggcaacccttgactgggagggagggtctcattgccaagggcctctgtgggaacccaaactgctggctccacacagtcctccaagtagacacatctctgtgtgacttcatccaggacctggggggtggggcacacagggacacagccttctaccctgggtacgtcccggcagctggctgcccgtgggtcccggcaggtttggaagcaggggctggcacaggcatcgtagcgccactcgcagatggggtaggcagcccccgagggcttggcatccagaaggcggaagagtgtgccccggcggaacacctctgtgtgttcgtacagccgcagggccagcaccgcgcccgacacatagaggaaggagctgggcttggccagggactccagggccaccaggcctgcctgccgtgtcccccggtgcagcaagaaggaggcatgctgttggaaggtgtcacggccctgccacttagccagctccagagacccgttggctgtgacgtgaaggaagaagttgggtctgtctgctgcctccagggacaccacatctgggtcatgggccttggccttgtacagagcagctgtcagcaggaagctcacaatgtctgctggcgccacatcctctgtcctcactaggactatgtcatcgcccaccgccttcatgcccaccagagcaccaccggctgccaagctggatagctgataggggcccttacctagcactttgttaaagaagtcacagtcatacgggcagaggcggggggttcgccagtcaacagccaccccatgctggcaacactggtgggcataagcggagacgctggcacagaagcactcacagtcaccaccctggctgcagccacatgtgtctgtcaggcagtttgagtaaaaccaagtgacatcaaccacagggtggcagatctcaaacacctcactgagcaggatgctgcactccttcttggcaaatggttctcggagaggattcaggacacacatatcccgaggatcgagggtgtctgggcactcaactgcagcccaactgctgccaaactcctgggggttagttagctctaggttctccggggtcctcatctcattgatggtttttaagtcaaagttcccacagaggcccgccagctggccctgccactgaggcccagcctggacgtgcactgtggttctctggtcccacaagagggtgatgtgctcctgtgggaaatgcaccagtgtgaaaaatcccactcgccatgtgtggacctcctgcttgtcatccaggaagctctctggactaggatttccggagtcatcatcaaagacaatgagtgagttcccaacgttgatggaaataaatttcctgcagatcatgccagagctgtagcagttcacattctctacaatcacagagaagctgacatctgatgtgctcttgaccaggtgcactttgcatgcccccacgaagtcaaacgggagcccatcaaacgtgcggtaatgccggtccccataggcagtgcaggtggaggcgcaagggtgcagggtgcactggaatgagccccgctggcacacacaggtatggcaaggagacatcacctggtccccagggaaatactccttccccttccaagtgcaggggcactcctctggcaggaaacatgcatccccgtgtctgagcagaccctggggacaggcgcagcccgagaggcaggggccacgggctgacacgctcaggttcagcagttgctgctcacacgtcctctccctgctcagctccaggtccgtgtgcaggtcgctgcagttcacgaagacctggcctgctgggcaggcagcagctggggctctgctatcacagctcatgactccatctttgcagtggcagtggcccagggatgggatgtcactgtctccggggggatagtccactccctggaagtggcaggagcactggttccgggggacacagaggtcagcctgggtgtccagataggtgtccggtgggcaggcacagccctccacacactcgtctctgctcaggtcatcgccaccatcaaccccacaggcctcagggctggccaggtcctggcaggtacgtccacacggggccacgcaggggctatactccttggaggcctcacaggacagtgcacaggctggcaggcgggcgcggaaatcaacggggagcccatggcgccggcacaggtgggcgtagtgggccagtgtggcgcacaggcagggctgcccgcagcggcaggcatccctgcggcactgctcaaagtagggcacggggctcaggaacgcagagcagggcgcaaacatctcccccgtgagcacgctgcaggcctgcactgagtaggaggcggcttgcaggtgcacatcgcaggggtccagaggggagccagagaccagcggggagcaagcagaaagtgttttccaggaattgccaaaaagttgtggggtgctctcaggtacacccactggagacaggaagtcatcctgcgtgttgccattgaaggtgccgcagaggcccacggtatcctccacccatcgctggtccacttgcaggtacagtcggagcccttcacggtcgtagagcacccgcacgcccacgttcgtcctcacccgcaggaacacggaggacagcctacggatctcaaaggcatcatctgtgtatggcgggatgatcttgtactggtcaaacagaaggacatcccctgcctgggtcagggtcacctgcctccgagggtcctggtgcagaatcactgacactgactggacacaggctccatcttggttcaggccacatggggcattctgcaatgtcacggtgaaggtgcccgaagagcggctcttggccaggatgtactgacatgtggcggggaacgtgtaccggcggccatcaaaggttgtgaagtgaatgtcaccagtcactgagcactcagctgggcagacagctgtgctgcactcccacttgcctgaggtgcatgtgcaagtattgcagtcttccttcaccacagagccaggtgggtacagagtcccgtgaaactcacagggacactcagctggtgccacgcagcccccatcctcgaagatgagcccattggggcaatagcagccgtccacacaggcgatctcactgtccacacaggatgcccggggatggcaggaggcagggcagcaggcgatgcactcattgtaggtaaaggccttctccttgcagtgcacagtgcattgccggagctgggtcctccagccttgcaagggccgccctgcctgggcacacgcccgggcatactccgccagtgcccggcaccaggtggctacatcacccattgattggcagagatcactggtacaactggctgtgaagggcagagggctgacgtaggcgtggcaggcgtcaaaggggggccgcagtagagcctcacactgctcgtacacgccctgcatggttcctgggttctgctgtaggcacggtgggcgaggcagggaggaagttgtgggccctggaggctggttaggggcctgctcctgccagctgtgcacaaactcaaccacgtcgtcagtcagcttcccagagctggtcaccagatcatccttggggtcagcattgttgttcccacacagcccatgggtccagcccagaagctctggactcatcttgatgtagacagccgaggcaccatcccaggccagtgtgaaggctgactgatgccgcacgatgacatagccggcaagctgctgcagacgcgcgctccccatgacatgtggcagttggaccctcatgcctccatgggtgacctccttggccagatggatctcctgctcacccacaaagaagaggctgacagccctggagcaggtgtagggtgaagagccacactgcgggtcattgtgtacctggatggagaagctctgtccctcgggctcatggcgacccaccagggtgtagctgccctttccggagaggtagtagtagagcccatcaaatgtctccacgtggtgctgcccccacgcccggcaaatgctgtccctctcagggccggcattgtacaccatctggcagcgcggtccagtggcattgaagcgtctgcagtcacagaaggctgggtgcacacactcgcctccattgaagcaggagaacaagtaggatggtgcacacttggcccgatggagccgcctttcccaggaagacatggccacggagtctggggcttcagcctgctggcctcccacgactgtagccttgtcccccatggcaagggtcgcctcctggtggctgctgctgggttgcccggctggctctggctgtggctctgcactgccccacagaacgggtgctgcggcgaggcgctgcacccgcagggactcggctgcctgctcaccccagggcagccagacacaaagcagccagcagagcgcagacgccaggactcccatagggacacgaggggaccggaggacttgagcgcagggccagcctcccgaggtgcctccccgggctaaggcagggtcacacctccactccgcagccgaggtccctcttgttctcat

SEQ ID NO: 9142 - RNA, 1018 nt, Homo sapiens
  source 1..1018: mol_type = other RNA
actgggcttggagtcagaagaactaggtgagagtttcagctgtgcctcttacctgcctgccagtgggcaattcatttttcctctcccaacagtcttctcagccatgaaaagaagtgacagcagtcactgcatggggttgctgtgaggactaagtgagagtgtggagctgaaatcctctgacaaactgtgcagtgctcttcagatgtcgggacctttgttgcagccctcacctactctccacctcggctgtgctttggaaacctgcccaggcaccagctatgtcgactcccgctgccattcaggcccataaggatatcccagaaaataattttgccacctctctatgttaacagctcgaaatctccagacacttctgattaccaggattttgagtacatgacggttttcttcctcaaaattcttaaatagcaaaaaggcttgaatgacagtcaggactggcagaagttggactgtcattgtgaaccaaggaaggaggcacagttggaaacccactgctgagcctccttccttttagcttgaaagtgctctagagtttctgagctcacaatgcatctctttggaagtctgccctcccagggttgccatggtgactattttggtactgcatgctagaaaaagccgaggcacctgctggtcacaccaccaaaacttgtctctctgaaaaatcagcagatggcatttgtcagaaattcctacttcttgattaatttgggaaaaagaagagtgtgtggcagtgctgatatcctttaacctggaccgggcgtgttggtgtttcagggaggatgtgaaaagctgtgcacagaccccatgaccttcttctgaagtggtgggtcatttagttttcccagagaggcaaagaagtttggtgatttggagcctgttggttctctatgaggaatgagcctcaagttccccactggcaattttgttctatcacaagtcctggtaagtcctggctgacaaattctgggtactctcctttcctgtggccatatca

SEQ ID NO: 9143 - RNA, 798 nt, Homo sapiens
  source 1..798: mol_type = other RNA
actgggtaggtggggctccaggatgggctctaatagcagcagccttgtctctccctgccccctgccctgccccaggggtcaaagggagctgggcggggcgcctaggaggttggcggcaactcttccccactctgccgcagacgcttcttggctctgatctcattcatagcctcttcaatggagcgtgtgtccctcttattggccacgggcacacagccgtaggtcttattggcctgtagcatgtgggctgcgtctttggctgctcccttgccgatgaggtggctgtacttgtccttgtagtcgctggcagggctcaccaccacaggcccctgctgggctgcctcctcctcttgcctctgggccagctccttcagcttccgcttctcctcagccttctgggggtcccattcctctccacgacggtaagagtctagctcttcatctgagggtgcaaactcctttttgaagatcatgacatagcgacagtcatcatcttccccaaaggagaaggatgtcaggccagccacttccaccacatcatgtagtatgctcctctcgatcttgttcattggctgaaactttttcttgatctgcccactgtcttgaatgaaatctgacacctccttctccatccttttacgaaactccactttctgttgtttctcttgctcttgtagtttcttcaggcgggcggcctgttctcgggccttgcgccgagtctcctggtcaccgaggctgggtggcttctccatggagctcaggatggagcccagtaggtccgccatcttgggagtgact

SEQ ID NO: 9144 - RNA, 1443 nt, Homo sapiens
  source 1..1443: mol_type = other RNA
actgggtaggtggggctccaggatgggctctaatagcagcagccttgtctctccctgccccctgccctgccccaggggtcaaagggagctgggcggggcgcctaggaggttggcggcaactcttccccactctgccgcagacgcttcttggctctgatctcattcatagcctcttcaatggagcgtgtgtccctcttattggccacgggcacacagccgtaggtcttattggcctgtagcatgtgggctgcgtctttggctgctcccttgccgatgaggtggctgtacttgtccttgtagtcgctggcagggctcaccaccacaggcccctgctgggctgcctcctcctcttgcctctgggccagctccttcagcttccgcttctcctcagccttctgggggtcccattcctctccacgacggtaagagtctagctcttcatctgagggtgcaaactcctttttgaagatcatgacatagcgacagtcatcatcttccccaaaggagaaggatgtcaggccagccacttccaccacatcatgtagtatgctcctctcgatcttgttcattggctgaaactttttcttgatctgcccactgtcttgaatgaaatctgacacctccttctccatccttttacgaaactccactttctgttgtttctcttgctcttgtagtttcttcaggcgggcggcctgttgtgtgatcactgcatcaatgagcgccccagccccggactgtggcctccctgaggggtacccctggtccctaacggttgttcaagaaacaaggggacgaagcgtaggcaaccagcggcccttgaatacttggaaggcgtcctgcctgctctggtccccctggggcacgtggggagctgggacagggctcgtccgtggtcaaggtccgcaggtttgggagttggggtcctgcgttccgccagtatcatcccaagctgcaacacgagcagccccggggaggctcccaccgccctgcagggccgcgccctacgccggccgccgaactccagcccacccgcagggaagctactccgagaacgcaggcggagacagtggccaatcggacccggcgggtattctcatccctccaatcaacactacgatccgcccgggcagctcgggaatttaaggctacggatgggaaaaaggttgtcggagggaggcagaagggactgggttaaattaagcaggaggggcaagaacacacagaggaccctgcaaccaatgggaattcgcaggctggggtggtttcgaaggaaggtcgaacaggcctgaggaggcagagctttaagttgagatagccaatagagatgaaggcacagtagatggcgtgtcctaaatccaatcgaaatagagctagaggtgagcggggcaggaatgcggcaggttggaggcaccctaccaatcagaccaggtcagcagcgga

SEQ ID NO: 9145 - RNA, 5222 nt, Homo sapiens
  source 1..5222: mol_type = other RNA
actgggtaggtggggctccaggccttcgcagtctgtggcttataaaatgtgcagaggccctccttccagaccctggggacgcgggagaggcctggctgcagctcacagcagccacagccaaccccactgcctcccaaggcactctgggtggatccgcacagctgcctgccaagccagcctgcccccatcctgtgcctgccttggtttcctttggaggacctggttgagttccaaaccagtttgaaactttgaagccttgctgcgtagaacgcacacaggaacccgggggcttggatttgaaaccctttccacttctggcctgtgatgagacagaggcagctggaggagcagcggcctcactgtccaccttgaggggccacggctctgtctgtggaaggggccccgactgagcccccatctgcggtgcttgaggggccttggccctgtctctgcctgctgaccctgccacccacgacagaaacaagcactgagcacccagccaggaggctcacaaagaggcctttatttatctagctcaaagtagacactatcacaatcttgtttgttactccttttactaaaatagttcaaatcaatgtttttaccacactatcaaaaagttctatttcttcttgtctccccacgtcagagtggttgaatagaaggtagaaacaggccgggagtccacgggctcccagctctaaacggcgccagggcaggaaggggtggctccaggtctcactgtggcaccttctacagaaaatagacgtagctgccgggcccggggacagaaaccagacgttccagtccatctccaaaaagcagcacaaatactttgccccacagtatgaaaaatatacacctctaccgctctgcagtcatgcatttagttttaagaaaaaaaaaaaatcagtagtatgtatcttgtttcctcaagtttcaagaaaaaaaaaatgaaaggtcacttttttctctttaaacactgatgtgtagctagtaacttggataaaaaggtgccaccctacaaaatgtgctcagcatgttctgaggccaggatgggcttggccacctgggctggggcgaaaggagacctccatctgtcacagtggaaactgaagccgagtgccagtgccgcgtccggcttcaagatcaagagtcagagcctttgaaatggaaagggggcatctgaaagggcacccccactgggggctttcagagctaaggctccagaaggaagggggtcgccctgctagtgacggagctgggagtcaccctgagctacagcatgcccagatttcccctgtgggaagccccatctgaccttctacagcccacggctctgcaactgccacctgtactcaggtacatggcgtcgctgctgctggcttttaaaatcagctattagtttgagatgtgacagtcgccgacagggttctgtcctagaaagccatcccagtgccgtgttggctcaggggtcaccagctttgtgctgcctccgtaacagcaggagggttctcaaagcaatgttccactgatccctggatgccactgcagcattaaagacagggtcagtccccttgaggggaaaggtggcttcaaggctgttctctgggcctgtttgcaggagatccgcaggtaccaggagcccgtacttattgcttatttcagtggtggccacgccaacctgacccaaacatgatgcacacgggctcccagacttggctgccactcaaaatggacccacagcccttgggctactctgcggttctttggactgcaagacccagaggggcctctgctcagctgcccactcgggcaagaatcactgggtaccatgagcagcaggtgttcacccaacttcacgtgtacacccctagtgaccgggagcgcaccacctgaccgggcgacactccttcccaaagagcctcctggcaacacccacggcaggagcgccacaccatcccatcaccagcacccacttacccccctggggctaagatggggggcgtgagcctttcccctgagagcaaacgggcagcaagaactgctcagaatagagccgccagctagggagagggacagggcggccatctccctcctcttgcctgcatccccagccctgggcctgcatgagacctgctgggtaggaagacagcctctctgggctcttcaggtggggctgagcagcccctggaagagcacaggagtctgacgaggacctggtgaggtcctggacccaagagctagggctgcttacagtggcatgagcggatgtggggaagcggcctgtccccgtgctgcagctgtgggatcaaaatccctgtcatgtgccacacatcaccccctctaggccttactttcctcacacacacagttttctattgcactttacagtttatacatggtcatttacactgaagatctcacttgatgccagaatcctgtgaggagggccttatgctgcccattttactactgaggacacgggctcagagtggggaggcaactctccacccgcagcgactgcaaggcagcagaactcagctccacccggcccgccctcagccgtcggctgttggctcacgccccctcagtgaggacccctgccctgtggcgctggatgacctggagccataagcatggccgaaaaggaacctcagagacctgtttccaccaagagcccagacaggctgagtgaactgctaaaggtcacaccacaaactaaaggcagaacctggccagacacgctccttcccaaaaagaacagaactctcatctgcagcctacacagctctgtccacagggacccaagatgcagccaggccctgggggaggtcacagccaaccagagccccagctgtggcccagtgctgcccatcaggaaaatcacatgtggctcagcccagaaactctccccaggcccttcctgttactggcctgtcatgtaaaccacgaaaagggacgtgcctcaggcatggggcaggaggagcccaagaagggcatagcctggacagggtggcagggggacattgcagagactgggggggagggggatgacctccaaaagcaaggagcagcgggcatcgggtggctgagcacagatccccaggtgtgagggcaccctgacctccaaggctgagggtcacaggaagggcccagggcagcctccagccagccacagatgtggtgagtggccttgtccacatgccggggacccagtgcttggggggcctggggccaggccacggcatttgggcaagaagtggtgccacctgcgtcaagacccaggtagtggtggtctctgtccagtgtgggtggcagccggggagtagagggtttgatgagtggcccctccatcccaggcaggacagaggagcctggacagttcccaggctggatctcagaagcagcctgcagcctcttgctcatggagcccagggcccagagggggaatgaggcgtccgggccgctctgctgcaggaacagtcgcagcgtctcgtcttcccaggttgctggtgtatgaggcgggagatggcggcttgggccagtgcatcggacccatggcagctgggccagggcgggcagcgtcctatgtacagttcaccacagaggaagaagacaggggctgggctggaggtcctgcccgtgtctggggcctgaaactccccctggggacccccagcagggccagtccacgtccacagaagagtggccctacaaaggccccttgaactggttcccagacaggtgctgccgtatggagggcttggagctggctgcatctcccagctttctccagaccacgttgcacatctcgcgaacgatggccttctccttctcactcaggtcctcctcacagctgtcctggagctgccggtccagattctcgtgtacctccaggaccttcatggcatgcacgacagcctcgggcttctgtcctgcagggctgtagccagcagaggggggcgagggcagctcaggtgcggggcaggccgggccgttctgcagggagtcctggtaggagggcggcagggacgcaagctgggactccgagtggtagggcgagaagcctttccgcagcgtgcggaactctccggagcctgcctgctgtgcgaggagcttgtcaccctccagcagcctcactttgctctccagttgcctgatgtaggtggatgagggatcgtgcaggccgttggggatgctgcggtggtgcggcggcgccgacaagtcgtccagggaccgacgtgtggctcctgccttgccgtcgggggccttgtgcggcccggggggcagcagcgggggtgggacgtggtggtggtggtcggggctgccgccgctgcccgcgctggacgtactgctgccgtcgcccacgtcgcgggcccccgcgccgggcgcgccacccgacagcggcccgctcaggctggcctggctgtcgatggagctgcgggagccggcgccgcccccgccgccgccgccaccgcttgcggcccccgtcgccgccagtgccgcgcgctcctcgtccagcagcagcaccagctccttgagctccaggttctcgcgcagcagggcctcctggcgcgcctcgagctcgcgcagcttctgctgcgagcgggccacctcgtgccacacggcgccggccgcgtggcgcccgaagcgctgccactcgcgcgccagcttgcgccccttctgccggtcgtcgtcgaggaagcagcagagctcgcgcagctcctggttgtcgtcctgcagccgctggttcacgtccttgaggccgcggatctccagcaggtgctgctgcagccgccggttcacgtcgcgcatcaggccgccgtgctccagcatgaggcccaccttctcgccctcggcgcgccgcagccgccgcgccagctcctccttgctccagcgcagcagctcctcgtccggcacctggctcagctcctccgacgccgccgccgccgtcgccgcgggcttagccatggcggggccgtcaccgcggcatcgccctcgccctcgcccggccggcgcttccccgcgccggggctccgctgggccggtccgcgcgcgggcggggggcggccgggggcgcgtgcggcccgccccgcgccgcctggcgcgtcctctcgccgcgcccgccggggccgcccgggagcccgcgcgcctcggggttgacgagcggaggcggctgctgcgtcggcggccgcggtgccgggcgctctcagggttct

SEQ ID NO: 9146 - RNA, 983 nt, Homo sapiens
  source 1..983: mol_type = other RNA
actgggtaggtggggctccaggtgttccatcgtaatttcttcccgggaccatccagccttgagcaactttaggaccacctcattgattatatcgcccctgagattactgagaaacagaaagatagtccatggagactcagccctgtggccctcaggggcccggcgttctaagtgtggcccaaggacctccagcagccctgggtgcagcttctccgcttcatcgaagatgaacagggtctggtggcagagctgctgcgtctcccggatctggctcatcagctgctccttgtacaggtccacatatttggggtgaggaaagtggaacgtggcgatgaacatcctgacacagtcactcatcagcccgtcccgatacaggttctccaccagcatccgtgccacgaagttcttgcctgtgccagaccagccgtggaacgacagagcaagggccttttctggctggggcgtctctaagtagcccctcactgttcttaggaccagctgctggaccaaatgctggccatgcagccgcacattcaggtcccactctaagcctgtaaagttgttggagattctgcaatcccctctagggcagcagtctttgaagctgcagtaccacgtggtcaggaggtccaggtaccgctggcccaacagaggaaggcgccagcccaggggccccgtggctgcctcctcgtcctcgtcacagtcgtcgggccacacctggcagctgaagagcgtccagtaccgcttggagagggcacccgccgccctgagctgctcctgcaggcgctggaagcccggccaggcccaggccgagcccggctcgtcggttccctcccacggcctggaggcgccgcggggctcaggcgcgcccgggagcagcagcaggaaaaagagccaaagctggcgccacggaccgcgaagcatggccggccccgagctgcgggaccatccggctgccggcctagccaggctcccttaagccc

SEQ ID NO: 9147 - RNA, 6381 nt, Homo sapiens
  source 1..6381: mol_type = other RNA
acttacagacaagagccttgctcataaacagaggctattagagagccacagacaccctgacccccagaggcccagaaaggctggattcacactcagaagtgaggccttccctgggtgacccacacacagcagggtctgcagggagtgtggtgtgcggaaatggcaagaggggtggagggctagggaagtcccatggatctgtggttggacagcctgaggccagctccactgtgtctgaggggggtggcaggggagggcacctggcaaggccagcccacgtgagggacaggaagctgactgagctaagaccagcacttggccctggggccagcttcccaaatgccacaagggccactaggaaagatatggtggggagtggggacaattctctcaaatctgagtcccttttcaattttcagactttttttgtttggttgttgctcaaagtaaaaatgcgaggaaagtatcctgtgtgtttgcatgtacgtgtgcaactgtgttttgtatcagttgtgtgtgggtctgtgtgtacgttttgtgttgtaggttgttcatggcatgtgtttgctgtgtatgtgtatcctgtgtattgtgtgtgcacatgtatcgtacatacgtgtgtatatgtgtgttgtgtgtgtgcaaggctcacagatataggagagtcagtgtacgtaaaggcacacctgtggggagaaggtgggcaggccgacttctttgtgctcagggctggctgtgggctggctgggggtggggaggagaagcttgttctggcccctgggtgtgggggtgcagaggagcacacccactggaggtcaccctgccctgggctcctgggagcaggggaggggcccagtgacaatgtagtgtgtttaagcctgagccaggctgcaaccttgcccagctcagctgtggtgccccagaggcccctgtggggacagtggccaaactacgtccacagctcagccaggtctcacctgtcagtgctggaacctgagcaccaagacctgcagcacctgcctggggtgtggcagggagagccctcacttgaggcaacttcaccacttaactctttacttgcccctgcccctcaacccgccagggcacctgcaccctcccctccaactacctcctcgtggatctggccagggcccttggtgtcttatccagcacacctgttgcccacctgcctgagggacagggaggtcatcctcagggtgcccaggacagatggtgctacccaggagaggcactggtactaacctggacagaccagctgcctggctgtgcacctggcccacctaagttaggtttctcagggtccctatctttgacccctttgatgacctccttcccttgaaaatccttctcccaggctctccccaccttccctttactcctccttgctcctttgcctcagggagatgtgaagccccctctctacccagatctgatcaaggaggttgggaacttgggaactgccacagggatggggtggggatggtgggggaagccctgtggtgctgcagcccggtcctgcatccttccccacccagctccatcatggcgtttcccacacctctgattggactggaaactccctgaaaggaggaagcaagtcagattcacctctaggtccctcccaggcctggagaggctggcatgctgttggcactcactgactgcctggtggccgactggctggatggaatggtgacctgtgaccagtctgtctctctcctcagctgatctgagagttcctggaggccagggactgtgtttgcctcacctcggcacctctgtgcctggggcagaggaactgctcaacaagttctggttgaacaaatggagggaacactaagagcgaataattattaagcgcttactgtgtgcgagcagctgctgtaagcaatggacactttatctcagtgaaccctgcagagggttccaatgagggaatggagcagacctgatctaaccaagctaggggtggggaggtgcccggtggtaggtgccagcagacatgacaggcactcccgcacatggcaccacagcaatgctgtcaaggttgcccgtggaatctgaaagctgaaacactcatctttatatacagagttggccaaagcaagacaccagcaaatcagtttacccaaaaatgtgcaaacaagatttcctgtgcctgcctgtctgcagtttttctttcccctctctcttatataactcttgttgaaatcagtctatagatacatgttccttgtacagaaataaacagagagctaataattagtgaaacgtctttgggttattctttgacatacatattaataacagccccctgagggaggattctattattgtctgcattttatagatgagaatgtggaggatcagagaggttaaataacttgcccaaggccacacagctggtaagtggggagagaagtatgccccaggcagccccacctgtccagactccatgacctaatgctccttcctttctcaggcatagcccaggaagggcagcagaaccaccctgaagtggctggagtgtgggtcacaccatctctgcacttccctgaggtgatcttgaggaaggatggctgatcctatgcctgcttctcactccctgggactgcactgaggccagagcctgtacccctcatactcagatcaccctctggagctcctcagggcctgcaggagaaggtgctgactcctctgtgttcagactctacatccagcccacccctcgctgtcacacactgtcccctccaagcacagaccctctctctcctggctctctgcctggccgttttccttcacaaggaaccagagaaaaactcttccttcccagagacccttaggaccccaccagaatcatcagttcatcccggtggcctttgctctaacttgctgtgggatctctagatccgtgtgaccccatgcagggtcaggggctccctgaggagtgggggccagctagggtccctccatagccccatccccaaggaaggggctgagaagacagggtcccaggagccgcagtggcttttccaaggaaggagctgacaagatgctcgcaggagccccagtggcttttcctggggaagggggtgttttcacagtatgtgcacctgcatttgtgcatcactgcacaagcaacacacaagtggctatgtcttcacgtgtgggaatgtgtgtccacatccacatgtgtgtgctcatctgcacctgtgtgtccatgagtgtgcacacatggaggtgcctgtgtgcacgtacagttgcatgctcctgaattgaggtatgtgtgtgcatctgcatctttgtgtggggctgtgggtgcacctgtgtggccagggtgtcggagttggggtgtgtggctatgagtgaccctccttggggccactccttcctgtagctataagtgcatagttacagctgagaaagggcaacactgacagtcatagaggcctgcggatcttagggtgcccctgcagcatccctccaagttcaccatggcgagggaggtgcactgtacctttgactggagccactacctcaaaacccttctgcctgaagctccagctgagccccacctcggccctctgccaccagcatccatcagcagtcttggtgagcaaacaaagatgcctcttggagctgctgcctaggggtggggttgttcagtggtgggtgggtgcgcctaccctgggtaatctctgaacggcaagaccctggttttggggtcaggcagactgcagttaaatattagctcagcttctttctgtgaacctcagtttcttcatctaggatgagggcgatgaacacctgcccgagggactgcatctgtccattcacagccgccttgccatcccagagctctcgcctctgccagtgggctgctgggcctccctgctgctgtaacccagccagcccagggtctcctgcagtgtcccaccagggcttctcttctgccttcctggcctgagacattggttttggtcatccttaaggagcctcttctggtagaagtggttgagctggctgccctgggctggcttcccggagcagatggagtcctcagacagagtcttatcctctcaagacctgaggctgcccacccggccaggccgacactgggctgtcatcctattgcttgcctgtcttctgctgccgcagggcctgcaggaagacacttttcacctggcccaggatctcatggtacatccggaagtcctcctcctttccccgcagggcactgcccagggcagcctttagcatttcattctcctccacctggatggccagcctggttgtcagctcttccatttgggattccacgggcacatcggagagctgggcaaaggatgggtccttcttctcgctcccggttgggttgtgcctgttgttagaggtgggcagacctgttttggtcctgggagctgctctctgggaggctgatgccttccctggctccaggcgtatcttctccagatgttgctccagcaccacggtgcggtgtcgctcctcctgcagcttcctctctgactccaggagcttgctgttgctctcctccacccgtttctgcaggacagtgacaaactcggtgagccggtcacgctccacctcggcagcctgccagagggccttgatctctgacacttgtgcctgccagcctttttgttctggggagtccgagaacctaggtgaggtcctgtggggactgggcagggaaggcctcgtgagagcagattccaccagtgtgtggcccaggctggtcacagagcgagaagatccaagcctgccaacatgatcgcctgctgaggccggggacttggtcaggcctgggtcctccaggaactgggtataggcagggctgacctcgcggccactggacccctcacccactcctttattccgaagatagtgcacattgagttgtccgatctccatctccagctgtcgcactttggcctcccgctcagctaccatggcctgcagctgggcgactaggctgttgctccgctgagcctcgctgttcagttgctggtccaggtggtgctgggacactcgcgttttctcctcctgcagactcaggctgcctaggatctcctgtagctgcttcagctggtccatgagggcgtcgatgagctcgtcatcatgccggcccttctccaccagggttcccatctgactcttgagggtcttcatctcacttgacagcagcttgttccgagacctcatgccctcgaacttcttttttagctcttcaagctctctctggaggacatcccgttcactggcaagtttctccaagccttcctgtttttccctttccaggctgcggatcctcagcaggtttttctcctgtgccgacagcttccttgggtctggatagacagacaactcatcactggctgttcccgcagactggctccgggcctggcccaattgcttctcaagctcttgaaccttgctctgcaaaacaagaatttgttgagcccgacccctccaggtccctggcgaagataggagctgctgaacgttgatgtcttccccaacctctctggccaaaaccttctgtgccatccgcagctcctgcttcacagactggatctggtttcggaggtcactcatcttcaagttggtggccaccagcctgtcctgcagggccttcacctctggggtctccagcaatgctctgtctcccatctgggccctcggtggcttggctcctgcgtcggtggcccccttggctgacagcctggtcagggctgtctgcagttcccgctccagctcctggatgcgattggtcagctgcttcaccctggtttttgcaccctctgattctgccatcaacagccggttcttttttgatagctccacaattttggtggcgaccacgtctccggctacaccggctgtccctgtgaaggcaaatctgtcctcttctattttctttttgaggtgtttgatttcaaagtccctttccttcagcagcttatacaatcgcccgttctcgtccaccgtttccctgagctcatttcgaaggtgttcaatctcatcttcaagcaccctcttctcaaagctatttttcgagtttggctcccctgcgtggagaaggctgaggccatctgaaacctccaagggctcctcttggtcgtcagctctgcttttgaggctcagttctttttccctctttttctccatctgcttctgtaaccgtttgtgctgcatctcctgcattgccttgaactggagccgcaaagtgttctgtgagctttcatctgctgccatcctgccagcggtctctctccacttctcccttctaggaccgcggcggctaggtcacctcctccggacgccgacacgcgctgccct

SEQ ID NO: 9148 - RNA, 6514 nt, Homo sapiens
  source 1..6514: mol_type = other RNA
acttacagacaagagccttgctcataaacagaggctattagagagccacagacaccctgacccccagaggcccagaaaggctggattcacactcagaagtgaggccttccctgggtgacccacacacagcagggtctgcagggagtgtggtgtgcggaaatggcaagaggggtggagggctagggaagtcccatggatctgtggttggacagcctgaggccagctccactgtgtctgaggggggtggcaggggagggcacctggcaaggccagcccacgtgagggacaggaagctgactgagctaagaccagcacttggccctggggccagcttcccaaatgccacaagggccactaggaaagatatggtggggagtggggacaattctctcaaatctgagtcccttttcaattttcagactttttttgtttggttgttgctcaaagtaaaaatgcgaggaaagtatcctgtgtgtttgcatgtacgtgtgcaactgtgttttgtatcagttgtgtgtgggtctgtgtgtacgttttgtgttgtaggttgttcatggcatgtgtttgctgtgtatgtgtatcctgtgtattgtgtgtgcacatgtatcgtacatacgtgtgtatatgtgtgttgtgtgtgtgcaaggctcacagatataggagagtcagtgtacgtaaaggcacacctgtggggagaaggtgggcaggccgacttctttgtgctcagggctggctgtgggctggctgggggtggggaggagaagcttgttctggcccctgggtgtgggggtgcagaggagcacacccactggaggtcaccctgccctgggctcctgggagcaggggaggggcccagtgacaatgtagtgtgtttaagcctgagccaggctgcaaccttgcccagctcagctgtggtgccccagaggcccctgtggggacagtggccaaactacgtccacagctcagccaggtctcacctgtcagtgctggaacctgagcaccaagacctgcagcacctgcctggggtgtggcagggagagccctcacttgaggcaacttcaccacttaactctttacttgcccctgcccctcaacccgccagggcacctgcaccctcccctccaactacctcctcgtggatctggccagggcccttggtgtcttatccagcacacctgttgcccacctgcctgagggacagggaggtcatcctcagggtgcccaggacagatggtgctacccaggagaggcactggtactaacctggacagaccagctgcctggctgtgcacctggcccacctaagttaggtttctcagggtccctatctttgacccctttgatgacctccttcccttgaaaatccttctcccaggctctccccaccttccctttactcctccttgctcctttgcctcagggagatgtgaagccccctctctacccagatctgatcaaggaggttgggaacttgggaactgccacagggatggggtggggatggtgggggaagccctgtggtgctgcagcccggtcctgcatccttccccacccagctccatcatggcgtttcccacacctctgattggactggaaactccctgaaaggaggaagcaagtcagattcacctctaggtccctcccaggcctggagaggctggcatgctgttggcactcactgactgcctggtggccgactggctggatggaatggtgacctgtgaccagtctgtctctctcctcagctgatctgagagttcctggaggccagggactgtgtttgcctcacctcggcacctctgtgcctggggcagaggaactgctcaacaagttctggttgaacaaatggagggaacactaagagcgaataattattaagcgcttactgtgtgcgagcagctgctgtaagcaatggacactttatctcagtgaaccctgcagagggttccaatgagggaatggagcagacctgatctaaccaagctaggggtggggaggtgcccggtggtaggtgccagcagacatgacaggcactcccgcacatggcaccacagcaatgctgtcaaggttgcccgtggaatctgaaagctgaaacactcatctttatatacagagttggccaaagcaagacaccagcaaatcagtttacccaaaaatgtgcaaacaagatttcctgtgcctgcctgtctgcagtttttctttcccctctctcttatataactcttgttgaaatcagtctatagatacatgttccttgtacagaaataaacagagagctaataattagtgaaacgtctttgggttattctttgacatacatattaataacagccccctgagggaggattctattattgtctgcattttatagatgagaatgtggaggatcagagaggttaaataacttgcccaaggccacacagctggtaagtggggagagaagtatgccccaggcagccccacctgtccagactccatgacctaatgctccttcctttctcaggcatagcccaggaagggcagcagaaccaccctgaagtggctggagtgtgggtcacaccatctctgcacttccctgaggtgatcttgaggaaggatggctgatcctatgcctgcttctcactccctgggactgcactgaggccagagcctgtacccctcatactcagatcaccctctggagctcctcagggcctgcaggagaaggtgctgactcctctgtgttcagactctacatccagcccacccctcgctgtcacacactgtcccctccaagcacagaccctctctctcctggctctctgcctggccgttttccttcacaaggaaccagagaaaaactcttccttcccagagacccttaggaccccaccagaatcatcagttcatcccggtggcctttgctctaacttgctgtgggatctctagatccgtgtgaccccatgcagggtcaggggctccctgaggagtgggggccagctagggtccctccatagccccatccccaaggaaggggctgagaagacagggtcccaggagccgcagtggcttttccaaggaaggagctgacaagatgctcgcaggagccccagtggcttttcctggggaagggggtgttttcacagtatgtgcacctgcatttgtgcatcactgcacaagcaacacacaagtggctatgtcttcacgtgtgggaatgtgtgtccacatccacatgtgtgtgctcatctgcacctgtgtgtccatgagtgtgcacacatggaggtgcctgtgtgcacgtacagttgcatgctcctgaattgaggtatgtgtgtgcatctgcatctttgtgtggggctgtgggtgcacctgtgtggccagggtgtcggagttggggtgtgtggctatgagtgaccctccttggggccactccttcctgtagctataagtgcatagttacagctgagaaagggcaacactgacagtcatagaggcctgcggatcttagggtgcccctgcagcatccctccaagttcaccatggcgagggaggtgcactgtacctttgactggagccactacctcaaaacccttctgcctgaagctccagctgagccccacctcggccctctgccaccagcatccatcagcagtcttggtgagcaaacaaagatgcctcttggagctgctgcctaggggtggggttgttcagtggtgggtgggtgcgcctaccctgggtaatctctgaacggcaagaccctggttttggggtcaggcagactgcagttaaatattagctcagcttctttctgtgaacctcagtttcttcatctgtcaaataagacaacaaacccctgggtcattagaggactgaatggggtcaggttgccacagtagatgctcactcactgggagctgcagtgattatgaaaatacttattattattacaagtccaagggtctgcacctgaggaagtgtcctgaggagtgggctgacaaactggttgagagcatagtgccccaagtctgtgtagggtgtggacggctacagatggagccgggatgggggtgaggggatagggcagggctgagtggcatgggggatatgcccacttagggtaaccaagggctcttctgtgtgtgaagccatggggacatccagggctagtacctaggatgagggcgatgaacacctgcccgagggactgcatctgtccattcacagccgccttgccatcccagagctctcgcctctgccagtgggctgctgggcctccctgctgctgtaacccagccagcccagggtctcctgcagtgtcccaccagggcttctcttctgccttcctggcctgagacattggttttggtcatccttaaggagcctcttctggtagaagtggttgagctggctgccctgggctggcttcccggagcagatggagtcctcagacagagtcttatcctctcaagacctgaggctgcccacccggccaggccgacactgggctgtcatcctattgcttgcctgtcttctgctgccgcagggcctgcaggaagacacttttcacctggcccaggatctcatggtacatccggaagtcctcctcctttccccgcagggcactgcccagggcagcctttagcatttcattctcctccacctggatggccagcctggttgtcagctcttccatttgggattccacgggcacatcggagagctgggcaaaggatgggtccttcttctcgctcccggttgggttgtgcctgttgttagaggtgggcagacctgttttggtcctgggagctgctctctgggaggctgatgccttccctggctccaggcgtatcttctccagatgttgctccagcaccacggtgcggtgtcgctcctcctgcagcttcctctctgactccaggagcttgctgttgctctcctccacccgagaagatccaagcctgccaacatgatcgcctgctgaggccggggacttggtcaggcctgggtcctccaggaactgggtataggcagggctgacctcgcggccactggacccctcacccactcctttattccgaagatagtgcacattgagttgtccgatctccatctccagctgtcgcactttggcctcccgctcagctaccatggcctgcagctgggcgactaggctgttgctccgctgagcctcgctgttcagttgctggtccaggtggtgctgggacactcgcgttttctcctcctgcagactcaggctgcctaggatctcctgtagctgcttcagctggtccatgagggcgtcgatgagctcgtcatcatgccggcccttctccaccagggttcccatctgactcttgagggtcttcatctcacttgacagcagcttgttccgagacctcatgccctcgaacttcttttttagctcttcaagctctctctggaggacatcccgttcactggcaagtttctccaagccttcctgtttttccctttccaggctgcggatcctcagcaggtttttctcctgtgccgacagcttccttgggtctggatagacagacaactcatcactggctgttcccgcagactggctccgggcctggcccaattgcttctcaagctcttgaaccttgctctgcaaaacaagaatttgttgagcccgacccctccaggtccctggcgaagataggagctgctgaacgttgatgtcttccccaacctctctggccaaaaccttctgtgccatccgcagctcctgcttcacagactggatctggtttcggaggtcactcatcttcaagttggtggccaccagcctgtcctgcagggccttcacctctggggtctccagcaatgctctgtctcccatctgggccctcggtggcttggctcctgcgtcggtggcccccttggctgacagcctggtcagggctgtctgcagttcccgctccagctcctggatgcgattggtcagctgcttcaccctggtttttgcaccctctgattctgccatcaacagccggttcttttttgatagctccacaattttggtggcgaccacgtctccggctacaccggctgtccctgtgaaggcaaatctgtcctcttctattttctttttgaggtgtttgatttcaaagtccctttccttcagcagcttatacaatcgcccgttctcgtccaccgtttccctgagctcatttcgaaggtgttcaatctcatcttcaagcaccctcttctcaaagctatttttcgagtttggctcccctgcgtggagaaggctgaggccatctgaaacctccaagggctcctcttggtcgtcagctctgcttttgaggctcagttctttttccctctttttctccatctgcttctgtaaccgtttgtgctgcatctcctgcattgccttgaactggagccgcaaagtgttctgtgagctttcatctgctgccatcctgccagcggtctctctccacttctcccttctaggaccgcggcggctaggtcacctcctccggacgccgacacgcgctgccct

SEQ ID NO: 9149 - RNA, 6732 nt, Homo sapiens
  source 1..6732: mol_type = other RNA
acttacagacaagagccttgctcataaacagaggctattagagagccacagacaccctgacccccagaggcccagaaaggctggattcacactcagaagtgaggccttccctgggtgacccacacacagcagggtctgcagggagtgtggtgtgcggaaatggcaagaggggtggagggctagggaagtcccatggatctgtggttggacagcctgaggccagctccactgtgtctgaggggggtggcaggggagggcacctggcaaggccagcccacgtgagggacaggaagctgactgagctaagaccagcacttggccctggggccagcttcccaaatgccacaagggccactaggaaagatatggtggggagtggggacaattctctcaaatctgagtcccttttcaattttcagactttttttgtttggttgttgctcaaagtaaaaatgcgaggaaagtatcctgtgtgtttgcatgtacgtgtgcaactgtgttttgtatcagttgtgtgtgggtctgtgtgtacgttttgtgttgtaggttgttcatggcatgtgtttgctgtgtatgtgtatcctgtgtattgtgtgtgcacatgtatcgtacatacgtgtgtatatgtgtgttgtgtgtgtgcaaggctcacagatataggagagtcagtgtacgtaaaggcacacctgtggggagaaggtgggcaggccgacttctttgtgctcagggctggctgtgggctggctgggggtggggaggagaagcttgttctggcccctgggtgtgggggtgcagaggagcacacccactggaggtcaccctgccctgggctcctgggagcaggggaggggcccagtgacaatgtagtgtgtttaagcctgagccaggctgcaaccttgcccagctcagctgtggtgccccagaggcccctgtggggacagtggccaaactacgtccacagctcagccaggtctcacctgtcagtgctggaacctgagcaccaagacctgcagcacctgcctggggtgtggcagggagagccctcacttgaggcaacttcaccacttaactctttacttgcccctgcccctcaacccgccagggcacctgcaccctcccctccaactacctcctcgtggatctggccagggcccttggtgtcttatccagcacacctgttgcccacctgcctgagggacagggaggtcatcctcagggtgcccaggacagatggtgctacccaggagaggcactggtactaacctggacagaccagctgcctggctgtgcacctggcccacctaagttaggtttctcagggtccctatctttgacccctttgatgacctccttcccttgaaaatccttctcccaggctctccccaccttccctttactcctccttgctcctttgcctcagggagatgtgaagccccctctctacccagatctgatcaaggaggttgggaacttgggaactgccacagggatggggtggggatggtgggggaagccctgtggtgctgcagcccggtcctgcatccttccccacccagctccatcatggcgtttcccacacctctgattggactggaaactccctgaaaggaggaagcaagtcagattcacctctaggtccctcccaggcctggagaggctggcatgctgttggcactcactgactgcctggtggccgactggctggatggaatggtgacctgtgaccagtctgtctctctcctcagctgatctgagagttcctggaggccagggactgtgtttgcctcacctcggcacctctgtgcctggggcagaggaactgctcaacaagttctggttgaacaaatggagggaacactaagagcgaataattattaagcgcttactgtgtgcgagcagctgctgtaagcaatggacactttatctcagtgaaccctgcagagggttccaatgagggaatggagcagacctgatctaaccaagctaggggtggggaggtgcccggtggtaggtgccagcagacatgacaggcactcccgcacatggcaccacagcaatgctgtcaaggttgcccgtggaatctgaaagctgaaacactcatctttatatacagagttggccaaagcaagacaccagcaaatcagtttacccaaaaatgtgcaaacaagatttcctgtgcctgcctgtctgcagtttttctttcccctctctcttatataactcttgttgaaatcagtctatagatacatgttccttgtacagaaataaacagagagctaataattagtgaaacgtctttgggttattctttgacatacatattaataacagccccctgagggaggattctattattgtctgcattttatagatgagaatgtggaggatcagagaggttaaataacttgcccaaggccacacagctggtaagtggggagagaagtatgccccaggcagccccacctgtccagactccatgacctaatgctccttcctttctcaggcatagcccaggaagggcagcagaaccaccctgaagtggctggagtgtgggtcacaccatctctgcacttccctgaggtgatcttgaggaaggatggctgatcctatgcctgcttctcactccctgggactgcactgaggccagagcctgtacccctcatactcagatcaccctctggagctcctcagggcctgcaggagaaggtgctgactcctctgtgttcagactctacatccagcccacccctcgctgtcacacactgtcccctccaagcacagaccctctctctcctggctctctgcctggccgttttccttcacaaggaaccagagaaaaactcttccttcccagagacccttaggaccccaccagaatcatcagttcatcccggtggcctttgctctaacttgctgtgggatctctagatccgtgtgaccccatgcagggtcaggggctccctgaggagtgggggccagctagggtccctccatagccccatccccaaggaaggggctgagaagacagggtcccaggagccgcagtggcttttccaaggaaggagctgacaagatgctcgcaggagccccagtggcttttcctggggaagggggtgttttcacagtatgtgcacctgcatttgtgcatcactgcacaagcaacacacaagtggctatgtcttcacgtgtgggaatgtgtgtccacatccacatgtgtgtgctcatctgcacctgtgtgtccatgagtgtgcacacatggaggtgcctgtgtgcacgtacagttgcatgctcctgaattgaggtatgtgtgtgcatctgcatctttgtgtggggctgtgggtgcacctgtgtggccagggtgtcggagttggggtgtgtggctatgagtgaccctccttggggccactccttcctgtagctataagtgcatagttacagctgagaaagggcaacactgacagtcatagaggcctgcggatcttagggtgcccctgcagcatccctccaagttcaccatggcgagggaggtgcactgtacctttgactggagccactacctcaaaacccttctgcctgaagctccagctgagccccacctcggccctctgccaccagcatccatcagcagtcttggtgagcaaacaaagatgcctcttggagctgctgcctaggggtggggttgttcagtggtgggtgggtgcgcctaccctgggtaatctctgaacggcaagaccctggttttggggtcaggcagactgcagttaaatattagctcagcttctttctgtgaacctcagtttcttcatctgtcaaataagacaacaaacccctgggtcattagaggactgaatggggtcaggttgccacagtagatgctcactcactgggagctgcagtgattatgaaaatacttattattattacaagtccaagggtctgcacctgaggaagtgtcctgaggagtgggctgacaaactggttgagagcatagtgccccaagtctgtgtagggtgtggacggctacagatggagccgggatgggggtgaggggatagggcagggctgagtggcatgggggatatgcccacttagggtaaccaagggctcttctgtgtgtgaagccatggggacatccagggctagtacctaggatgagggcgatgaacacctgcccgagggactgcatctgtccattcacagccgccttgccatcccagagctctcgcctctgccagtgggctgctgggcctccctgctgctgtaacccagccagcccagggtctcctgcagtgtcccaccagggcttctcttctgccttcctggcctgagacattggttttggtcatccttaaggagcctcttctggtagaagtggttgagctggctgccctgggctggcttcccggagcagatggagtcctcagacagagtcttatcctctcaagacctgaggctgcccacccggccaggccgacactgggctgtcatcctattgcttgcctgtcttctgctgccgcagggcctgcaggaagacacttttcacctggcccaggatctcatggtacatccggaagtcctcctcctttccccgcagggcactgcccagggcagcctttagcatttcattctcctccacctggatggccagcctggttgtcagctcttccatttgggattccacgggcacatcggagagctgggcaaaggatgggtccttcttctcgctcccggttgggttgtgcctgttgttagaggtgggcagacctgttttggtcctgggagctgctctctgggaggctgatgccttccctggctccaggcgtatcttctccagatgttgctccagcaccacggtgcggtgtcgctcctcctgcagcttcctctctgactccaggagcttgctgttgctctcctccacccgtttctgcaggacagtgacaaactcggtgagccggtcacgctccacctcggcagcctgccagagggccttgatctctgacacttgtgcctgccagcctttttgttctggggagtccgagaacctaggtgaggtcctgtggggactgggcagggaaggcctcgtgagagcagattccaccagtgtgtggcccaggctggtcacagagcgagaagatccaagcctgccaacatgatcgcctgctgaggccggggacttggtcaggcctgggtcctccaggaactgggtataggcagggctgacctcgcggccactggacccctcacccactcctttattccgaagatagtgcacattgagttgtccgatctccatctccagctgtcgcactttggcctcccgctcagctaccatggcctgcagctgggcgactaggctgttgctccgctgagcctcgctgttcagttgctggtccaggtggtgctgggacactcgcgttttctcctcctgcagactcaggctgcctaggatctcctgtagctgcttcagctggtccatgagggcgtcgatgagctcgtcatcatgccggcccttctccaccagggttcccatctgactcttgagggtcttcatctcacttgacagcagcttgttccgagacctcatgccctcgaacttcttttttagctcttcaagctctctctggaggacatcccgttcactggcaagtttctccaagccttcctgtttttccctttccaggctgcggatcctcagcaggtttttctcctgtgccgacagcttccttgggtctggatagacagacaactcatcactggctgttcccgcagactggctccgggcctggcccaattgcttctcaagctcttgaaccttgctctgcaaaacaagaatttgttgagcccgacccctccaggtccctggcgaagataggagctgctgaacgttgatgtcttccccaacctctctggccaaaaccttctgtgccatccgcagctcctgcttcacagactggatctggtttcggaggtcactcatcttcaagttggtggccaccagcctgtcctgcagggccttcacctctggggtctccagatcacggcctcctgaagccccaagcagagggaagggtgttcagctccactctggaatgtgctttggaggcctagggttggaatgtggattgagcctgcaggcctctggagtgtggctcgggcttgggccgccctgagcagcctatgaggggaaacattgcttttgctctcgctctgatcaggagatgccagggagaacacgtggtgctgatgaattgagacctgcggcccatcacacactcttctctcagaacctggaacctcccaggctccctgtggccacagaataaagtcaaaactcctgctccagctgccattcaagggctccctctatgggtgacttcaccccagcttttttggctttcgttccccttttctcccgtgtgagctctgggctgcagtcaaatgttatccagctgacactcagttcaccttccccatcttccttctccagtaaggccagctcagggacgccctcctccgtcccaccttccagctgcaaccttaatggagggtggactcccctgtgagcttagagcaccggggccatctctgaaggccctgtccacatcctgccttcgaatgacttctcattcctcctctgggattctccatagacagagcctctgtttttttggtggttgttgtagttgtttgtttgtttgttttgagacacagtctcactctgtcacccaggct

SEQ ID NO: 9150 - RNA, 6119 nt, Homo sapiens
  source 1..6119: mol_type = other RNA
acttacagacaagagccttgctcataaacagaggctattagagagccacagacaccctgacccccagaggcccagaaaggctggattcacactcagaagtgaggccttccctgggtgacccacacacagcagggtctgcagggagtgtggtgtgcggaaatggcaagaggggtggagggctagggaagtcccatggatctgtggttggacagcctgaggccagctccactgtgtctgaggggggtggcaggggagggcacctggcaaggccagcccacgtgagggacaggaagctgactgagctaagaccagcacttggccctggggccagcttcccaaatgccacaagggccactaggaaagatatggtggggagtggggacaattctctcaaatctgagtcccttttcaattttcagactttttttgtttggttgttgctcaaagtaaaaatgcgaggaaagtatcctgtgtgtttgcatgtacgtgtgcaactgtgttttgtatcagttgtgtgtgggtctgtgtgtacgttttgtgttgtaggttgttcatggcatgtgtttgctgtgtatgtgtatcctgtgtattgtgtgtgcacatgtatcgtacatacgtgtgtatatgtgtgttgtgtgtgtgcaaggctcacagatataggagagtcagtgtacgtaaaggcacacctgtggggagaaggtgggcaggccgacttctttgtgctcagggctggctgtgggctggctgggggtggggaggagaagcttgttctggcccctgggtgtgggggtgcagaggagcacacccactggaggtcaccctgccctgggctcctgggagcaggggaggggcccagtgacaatgtagtgtgtttaagcctgagccaggctgcaaccttgcccagctcagctgtggtgccccagaggcccctgtggggacagtggccaaactacgtccacagctcagccaggtctcacctgtcagtgctggaacctgagcaccaagacctgcagcacctgcctggggtgtggcagggagagccctcacttgaggcaacttcaccacttaactctttacttgcccctgcccctcaacccgccagggcacctgcaccctcccctccaactacctcctcgtggatctggccagggcccttggtgtcttatccagcacacctgttgcccacctgcctgagggacagggaggtcatcctcagggtgcccaggacagatggtgctacccaggagaggcactggtactaacctggacagaccagctgcctggctgtgcacctggcccacctaagttaggtttctcagggtccctatctttgacccctttgatgacctccttcccttgaaaatccttctcccaggctctccccaccttccctttactcctccttgctcctttgcctcagggagatgtgaagccccctctctacccagatctgatcaaggaggttgggaacttgggaactgccacagggatggggtggggatggtgggggaagccctgtggtgctgcagcccggtcctgcatccttccccacccagctccatcatggcgtttcccacacctctgattggactggaaactccctgaaaggaggaagcaagtcagattcacctctaggtccctcccaggcctggagaggctggcatgctgttggcactcactgactgcctggtggccgactggctggatggaatggtgacctgtgaccagtctgtctctctcctcagctgatctgagagttcctggaggccagggactgtgtttgcctcacctcggcacctctgtgcctggggcagaggaactgctcaacaagttctggttgaacaaatggagggaacactaagagcgaataattattaagcgcttactgtgtgcgagcagctgctgtaagcaatggacactttatctcagtgaaccctgcagagggttccaatgagggaatggagcagacctgatctaaccaagctaggggtggggaggtgcccggtggtaggtgccagcagacatgacaggcactcccgcacatggcaccacagcaatgctgtcaaggttgcccgtggaatctgaaagctgaaacactcatctttatatacagagttggccaaagcaagacaccagcaaatcagtttacccaaaaatgtgcaaacaagatttcctgtgcctgcctgtctgcagtttttctttcccctctctcttatataactcttgttgaaatcagtctatagatacatgttccttgtacagaaataaacagagagctaataattagtgaaacgtctttgggttattctttgacatacatattaataacagccccctgagggaggattctattattgtctgcattttatagatgagaatgtggaggatcagagaggttaaataacttgcccaaggccacacagctggtaagtggggagagaagtatgccccaggcagccccacctgtccagactccatgacctaatgctccttcctttctcaggcatagcccaggaagggcagcagaaccaccctgaagtggctggagtgtgggtcacaccatctctgcacttccctgaggtgatcttgaggaaggatggctgatcctatgcctgcttctcactccctgggactgcactgaggccagagcctgtacccctcatactcagatcaccctctggagctcctcagggcctgcaggagaaggtgctgactcctctgtgttcagactctacatccagcccacccctcgctgtcacacactgtcccctccaagcacagaccctctctctcctggctctctgcctggccgttttccttcacaaggaaccagagaaaaactcttccttcccagagacccttaggaccccaccagaatcatcagttcatcccggtggcctttgctctaacttgctgtgggatctctagatccgtgtgaccccatgcagggtcaggggctccctgaggagtgggggccagctagggtccctccatagccccatccccaaggaaggggctgagaagacagggtcccaggagccgcagtggcttttccaaggaaggagctgacaagatgctcgcaggagccccagtggcttttcctggggaagggggtgttttcacagtatgtgcacctgcatttgtgcatcactgcacaagcaacacacaagtggctatgtcttcacgtgtgggaatgtgtgtccacatccacatgtgtgtgctcatctgcacctgtgtgtccatgagtgtgcacacatggaggtgcctgtgtgcacgtacagttgcatgctcctgaattgaggtatgtgtgtgcatctgcatctttgtgtggggctgtgggtgcacctgtgtggccagggtgtcggagttggggtgtgtggctatgagtgaccctccttggggccactccttcctgtagctataagtgcatagttacagctgagaaagggcaacactgacagtcatagaggcctgcggatcttagggtgcccctgcagcatccctccaagttcaccatggcgagggaggtgcactgtacctttgactggagccactacctcaaaacccttctgcctgaagctccagctgagccccacctcggccctctgccaccagcatccatcagcagtcttggtgagcaaacaaagatgcctcttggagctgctgcctaggggtggggttgttcagtggtgggtgggtgcgcctaccctgggtaatctctgaacggcaagaccctggttttggggtcaggcagactgcagttaaatattagctcagcttctttctgtgaacctcagtttcttcatctgtcaaataagacaacaaacccctgggtcattagaggactgaatggggtcaggttgccacagtagatgctcactcactgggagctgcagtgattatgaaaatacttattattattacaagtccaagggtctgcacctgaggaagtgtcctgaggagtgggctgacaaactggttgagagcatagtgccccaagtctgtgtagggtgtggacggctacagatggagccgggatgggggtgaggggatagggcagggctgagtggcatgggggatatgcccacttagggtaaccaagggctcttctgtgtgtgaagccatggggacatccagggctagtacctaggatgagggcgatgaacacctgcccgagggactgcatctgtccattcacagccgccttgccatcccagagctctcgcctctgccagtgggctgctgggcctccctgctgctgtaacccagccagcccagggtctcctgcagtgtcccaccagggcttctcttctgccttcctggcctgagacattggttttggtcatccttaaggagcctcttctggtagaagtggttgagctggctgccctgggctggcttcccggagcagatggagtcctcagacagagtcttatcctctcaagacctgaggctgcccacccggccaggccgacactgggctgtcatcctattgcttgcctgtcttctgctgccgcagggcctgcaggaagacacttttcacctggcccaggatctcatggtacatccggaagtcctcctcctttccccgcagggcactgcccagggcagcctttagcatttcattctcctccacctggatggccagcctggttgtcagctcttccatttgggattccacgggcacatcggagagctgggcaaaggatgggtccttcttctcgctcccggttgggttgtgcctgttgttagaggtgggcagacctgttttggtcctgggagctgctctctgggaggctgatgccttccctggctccaggcgtatcttctccagatgttgctccagcaccacggtgcggtgtcgctcctcctgcagcttcctctctgactccaggagcttgctgttgctctcctccacccgtttctgcaggacagtgacaaactcggtgagccggtcacgctccacctcggcagcctgccagagggccttgatctctgacacttgtgcctgccagcctttttgttctggggagtccgagaacctaggtgaggtcctgtggggactgggcagggaaggcctcgtgagagcagattccaccagtgtgtggcccaggctggtcacagagcgagaagatccaagcctgccaacatgatcgcctgctgaggccggggacttggtcaggcctgggtcctccaggaactgggtataggcagggctgacctcgcggccactggacccctcacccactcctttattccgaagatagtgcacattgagttgtccgatctccatctccagctgtcgcactttggcctcccgctcagctaccatggcctgcagctgggcgactaggctgttgctccgctgagcctcgctgttcagttgctggtccaggtggtgctgggacactcgcgttttctcctcctgcagactcaggctgcctaggatctcctgtagctgcttcagctggtccatgagggcgtcgatgagctcgtcatcatgccggcccttctccaccagggttcccatctgactcttgagggtcttcatctcacttgacagcagcttgttccgagacctcatgccctcgaacttcttttttagctcttcaagctctctctggaggacatcccgttcactggcaagtttctccaagccttcctgtttttccctttccaggctgcggatcctcagcaggtttttctcctgtgccgacagcttccttgggtctggatagacagacaactcatcactggctgttcccgcagactggctccgggcctggcccaattgcttctcaagctcttgaaccttgctctgcaaaacaagaatttgttgagcccgacccctccaggtccctggcgaagataggagctgctgaacgttgatgtcttccccaacctctctggccaaaaccttctgtgccatccgcagctcctgcttcacagactggatctggtttcggaggtcactcatcttcaagttggtggccaccagcctgtcctgcagggccttcacctctggggtctccagctgtggaggaggggaggcccaggcccatggctgcctcacagacttcccagcacagaagagaattcataccaatgctctgtctccc

SEQ ID NO: 9151 - RNA, 6598 nt, Homo sapiens
  source 1..6598: mol_type = other RNA
acttacagacaagagccttgctcataaacagaggctattagagagccacagacaccctgacccccagaggcccagaaaggctggattcacactcagaagtgaggccttccctgggtgacccacacacagcagggtctgcagggagtgtggtgtgcggaaatggcaagaggggtggagggctagggaagtcccatggatctgtggttggacagcctgaggccagctccactgtgtctgaggggggtggcaggggagggcacctggcaaggccagcccacgtgagggacaggaagctgactgagctaagaccagcacttggccctggggccagcttcccaaatgccacaagggccactaggaaagatatggtggggagtggggacaattctctcaaatctgagtcccttttcaattttcagactttttttgtttggttgttgctcaaagtaaaaatgcgaggaaagtatcctgtgtgtttgcatgtacgtgtgcaactgtgttttgtatcagttgtgtgtgggtctgtgtgtacgttttgtgttgtaggttgttcatggcatgtgtttgctgtgtatgtgtatcctgtgtattgtgtgtgcacatgtatcgtacatacgtgtgtatatgtgtgttgtgtgtgtgcaaggctcacagatataggagagtcagtgtacgtaaaggcacacctgtggggagaaggtgggcaggccgacttctttgtgctcagggctggctgtgggctggctgggggtggggaggagaagcttgttctggcccctgggtgtgggggtgcagaggagcacacccactggaggtcaccctgccctgggctcctgggagcaggggaggggcccagtgacaatgtagtgtgtttaagcctgagccaggctgcaaccttgcccagctcagctgtggtgccccagaggcccctgtggggacagtggccaaactacgtccacagctcagccaggtctcacctgtcagtgctggaacctgagcaccaagacctgcagcacctgcctggggtgtggcagggagagccctcacttgaggcaacttcaccacttaactctttacttgcccctgcccctcaacccgccagggcacctgcaccctcccctccaactacctcctcgtggatctggccagggcccttggtgtcttatccagcacacctgttgcccacctgcctgagggacagggaggtcatcctcagggtgcccaggacagatggtgctacccaggagaggcactggtactaacctggacagaccagctgcctggctgtgcacctggcccacctaagttaggtttctcagggtccctatctttgacccctttgatgacctccttcccttgaaaatccttctcccaggctctccccaccttccctttactcctccttgctcctttgcctcagggagatgtgaagccccctctctacccagatctgatcaaggaggttgggaacttgggaactgccacagggatggggtggggatggtgggggaagccctgtggtgctgcagcccggtcctgcatccttccccacccagctccatcatggcgtttcccacacctctgattggactggaaactccctgaaaggaggaagcaagtcagattcacctctaggtccctcccaggcctggagaggctggcatgctgttggcactcactgactgcctggtggccgactggctggatggaatggtgacctgtgaccagtctgtctctctcctcagctgatctgagagttcctggaggccagggactgtgtttgcctcacctcggcacctctgtgcctggggcagaggaactgctcaacaagttctggttgaacaaatggagggaacactaagagcgaataattattaagcgcttactgtgtgcgagcagctgctgtaagcaatggacactttatctcagtgaaccctgcagagggttccaatgagggaatggagcagacctgatctaaccaagctaggggtggggaggtgcccggtggtaggtgccagcagacatgacaggcactcccgcacatggcaccacagcaatgctgtcaaggttgcccgtggaatctgaaagctgaaacactcatctttatatacagagttggccaaagcaagacaccagcaaatcagtttacccaaaaatgtgcaaacaagatttcctgtgcctgcctgtctgcagtttttctttcccctctctcttatataactcttgttgaaatcagtctatagatacatgttccttgtacagaaataaacagagagctaataattagtgaaacgtctttgggttattctttgacatacatattaataacagccccctgagggaggattctattattgtctgcattttatagatgagaatgtggaggatcagagaggttaaataacttgcccaaggccacacagctggtaagtggggagagaagtatgccccaggcagccccacctgtccagactccatgacctaatgctccttcctttctcaggcatagcccaggaagggcagcagaaccaccctgaagtggctggagtgtgggtcacaccatctctgcacttccctgaggtgatcttgaggaaggatggctgatcctatgcctgcttctcactccctgggactgcactgaggccagagcctgtacccctcatactcagatcaccctctggagctcctcagggcctgcaggagaaggtgctgactcctctgtgttcagactctacatccagcccacccctcgctgtcacacactgtcccctccaagcacagaccctctctctcctggctctctgcctggccgttttccttcacaaggaaccagagaaaaactcttccttcccagagacccttaggaccccaccagaatcatcagttcatcccggtggcctttgctctaacttgctgtgggatctctagatccgtgtgaccccatgcagggtcaggggctccctgaggagtgggggccagctagggtccctccatagccccatccccaaggaaggggctgagaagacagggtcccaggagccgcagtggcttttccaaggaaggagctgacaagatgctcgcaggagccccagtggcttttcctggggaagggggtgttttcacagtatgtgcacctgcatttgtgcatcactgcacaagcaacacacaagtggctatgtcttcacgtgtgggaatgtgtgtccacatccacatgtgtgtgctcatctgcacctgtgtgtccatgagtgtgcacacatggaggtgcctgtgtgcacgtacagttgcatgctcctgaattgaggtatgtgtgtgcatctgcatctttgtgtggggctgtgggtgcacctgtgtggccagggtgtcggagttggggtgtgtggctatgagtgaccctccttggggccactccttcctgtagctataagtgcatagttacagctgagaaagggcaacactgacagtcatagaggcctgcggatcttagggtgcccctgcagcatccctccaagttcaccatggcgagggaggtgcactgtacctttgactggagccactacctcaaaacccttctgcctgaagctccagctgagccccacctcggccctctgccaccagcatccatcagcagtcttggtgagcaaacaaagatgcctcttggagctgctgcctaggggtggggttgttcagtggtgggtgggtgcgcctaccctgggtaatctctgaacggcaagaccctggttttggggtcaggcagactgcagttaaatattagctcagcttctttctgtgaacctcagtttcttcatctgtcaaataagacaacaaacccctgggtcattagaggactgaatggggtcaggttgccacagtagatgctcactcactgggagctgcagtgattatgaaaatacttattattattacaagtccaagggtctgcacctgaggaagtgtcctgaggagtgggctgacaaactggttgagagcatagtgccccaagtctgtgtagggtgtggacggctacagatggagccgggatgggggtgaggggatagggcagggctgagtggcatgggggatatgcccacttagggtaaccaagggctcttctgtgtgtgaagccatggggacatccagggctagtacctaggatgagggcgatgaacacctgcccgagggactgcatctgtccattcacagccgccttgccatcccagagctctcgcctctgccagtgggctgctgggcctccctgctgctgtaacccagccagcccagggtctcctgcagtgtcccaccagggcttctcttctgccttcctggcctgagacattggttttggtcatccttaaggagcctcttctggtagaagtggttgagctggctgccctgggctggcttcccggagcagatggagtcctcagacagagtcttatcctctcaagacctgaggctgcccacccggccaggccgacactgggctgtcatcctattgcttgcctgtcttctgctgccgcagggcctgcaggaagacacttttcacctggcccaggatctcatggtacatccggaagtcctcctcctttccccgcagggcactgcccagggcagcctttagcatttcattctcctccacctggatggccagcctggttgtcagctcttccatttgggattccacgggcacatcggagagctgggcaaaggatgggtccttcttctcgctcccggttgggttgtgcctgttgttagaggtgggcagacctgttttggtcctgggagctgctctctgggaggctgatgccttccctggctccaggcgtatcttctccagatgttgctccagcaccacggtgcggtgtcgctcctcctgcagcttcctctctgactccaggagcttgctgttgctctcctccaccctaggtgaggtcctgtggggactgggcagggaaggcctcgtgagagcagattccaccagtgtgtggcccaggctggtcacagagcgagaagatccaagcctgccaacatgatcgcctgctgaggccggggacttggtcaggcctgggtcctccaggaactgggtataggcagggctgacctcgcggccactggacccctcacccactcctttattccgaagatagtgcacattgagttgtccgatctccatctccagctgtcgcactttggcctcccgctcagctaccatggcctgcagctgggcgactaggctgttgctccgctgagcctcgctgttcagttgctggtccaggtggtgctgggacactcgcgttttctcctcctgcagactcaggctgcctaggatctcctgtagctgcttcagctggtccatgagggcgtcgatgagctcgtcatcatgccggcccttctccaccagggttcccatctgactcttgagggtcttcatctcacttgacagcagcttgttccgagacctcatgccctcgaacttcttttttagctcttcaagctctctctggaggacatcccgttcactggcaagtttctccaagccttcctgtttttccctttccaggctgcggatcctcagcaggtttttctcctgtgccgacagcttccttgggtctggatagacagacaactcatcactggctgttcccgcagactggctccgggcctggcccaattgcttctcaagctcttgaaccttgctctgcaaaacaagaatttgttgagcccgacccctccaggtccctggcgaagataggagctgctgaacgttgatgtcttccccaacctctctggccaaaaccttctgtgccatccgcagctcctgcttcacagactggatctggtttcggaggtcactcatcttcaagttggtggccaccagcctgtcctgcagggccttcacctctggggtctccagcaatgctctgtctcccatctgggccctcggtggcttggctcctgcgtcggtggcccccttggctgacagcctggtcagggctgtctgcagttcccgctccagctcctggatgcgattggtcagctgcttcaccctggtttttgcaccctctgattctgccatcaacagccggttcttttttgatagctccacaattttggtggcgaccacgtctccggctacaccggctgtccctgtgaaggcaaatctgtcctcttctattttctttttgaggtgtttgatttcaaagtccctttccttcagcagcttatacaatcgcccgttctcgtccaccgtttccctgagctcatttcgaaggtgttcaatctcatcttcaagcaccctcttctcaaagctatttttcgagtttggctcccctgcgtggagaaggctgaggccatctgaaacctccaagggctcctcttggtcgtcagctctgcttttgaggctcagttctttttccctctttttctccatctgcttctgtaaccgtttgtgctgcatctcctgcattgccttgaactggagccgcaaagtgttctgtgagctttcatctgctgccatcctgccagcggtctctctccacttctcccttctaggaccgcggcggctaggtcacctcctccggacgccgacacgcgctgccct

SEQ ID NO: 9152 - RNA, 9765 nt, Homo sapiens
  source 1..9765: mol_type = other RNA
actttaacatggaagtgctttcccccttaaagtttgttaccaatctgagtaattttgtcaattgatacttctgctatcatgagtaatgtttccatatctttaggagctattttaaattctttttctgtattctaccacctgtcaaatcctttgctcatttttcctttgagaccttagaatttttctcttcgatttgtagaagctattttttgaaaataagaaattaactatttggctgtgatattcattgcaattctttttccagtgtgttgtttcttgaccttttatgctgtttttggtacagagataattttgtttaaaatagtcaatattttccttcctggtttctgattgagggccatacttagaccttccccatgctgagattattatttttttaagtgctacttcttcttcatgcacttccatgattccatatttttacttttaaaaacttggtcctcctggaatttattttggtatctagtctggcatatggcccaagcttaattttttttagctgggtgacagagttgttcatcatatattgaataatccatctttccccaattaacttgaatttaacatataaagttaacataacttaactttaacatatgctgttaatacatttcaacatgtattttaaatttatttttggccatttcatcttgttccattgaccctccacatatcagcaccacattgttttaattattgtagctttataagatgttttaatatttggtcatgctgactcactcaggtttcttcttttctagatttttcttggatattcttgcctcgtagtttccaataatttttttttttttgagacagggtctcactctggctgcccagactggagtgcagtgatgtgattttggctcactacagcctcgacctcccaaggcttgggtgattctcccacctcagcctcccgagtagctaggactataggtgcacaccaccacacccagctaatttcttgcattttaaatagagacgggatttcaccatgttgtccaggctggtctggaactcctggactcaggcaatccacctgcctcggcctctcaaagtgctgggattacaggagtgagccaccatgcttggccttcattaaattttaaaatcatttcaatgctattggggaaaacctgttggcatttttattgggattacactgaatttatagattaacagtgaaaattgatatatttataatttttaatcttcttatccaaaaacgtggtctgctttttatctgtttaagttcttttttgtgctctttagtttcattgtatagttttattgttgcagaacttatattttcttgttgcagttattcttaattattttatctttttgttggaattataatatggctttttctttcatcgtattttctaactacatgtagtctgacataataggcaattagaaaataatatgtatagacttaaccttatgtttcactaatttatttgttctcctttccttcttaaaaccactactttcttctcaattcattttttcttgttatagtacgttattcatatactcttgctaatagcccatccctatatgaatagtttttctgacttggaacaagtaggaagttttttaaaaatcacttatagtccatccctgtatgaagatgaatactataagtacattattcctacttgttccaagtcagaaaatctatttattttgccctcgactctgaatgatagtttggggagagaagtctaggtttgatgttgtttttccacagcagtttgaatatgctacctgtattctgcttacgtctacccttgctagtgaaatagttattgtcaaattcacacttctttttgtagattttccaaactttttcttttaggattaaaaaagaatctttgatgttctgaatcttgattgtaatgtgttatgcttgacctatatattctgccactattctggaaactcttttagtcaaaagaggtatggtggtggtgattttaccccccaagggacatttggcgatgtctggagacatttttggttgtcacaactgacaaccaaccctggggtaggggagggagggtggtggatttgctactggcgtctagggagtagggccaaggatgctgctaaacatcctacagtgcatagagaagcctctcacaataaatggttgtccagcccaaaaagccagcagtgccaatgctgacaaaccctgaggtatgggttttttagttctaggctttggtctggccaactgggggcaaaatgaatttggcttcagcctcagggcaacactttctggctgggagattctgtcctggctttgtgacaacggttgtcctggcctgtggtggtgccagcctcagtgtattaccgtggtttacctagattttccctacctgtaccaatgactcataggttttagttcatggagaggcgcttttcttggttgtgaggatggctatgcatatggcaatgttttgaaatatcttccccattatttctatgagtttgttttagtagagggcgatttcagcatgtgaccttcaaggtctttatgcaaaggggcaaagtcaataaaattaattctagcaatactgaaagagaaaaggaagcaataaatcactcataaactcatcaactagaaatattcaaggttaataatattccagaaagcttttaaaaatatatcagagaaaatataagaacagctagatagaattatgttaaatcgaaggatatgatacataatattttaaaattatttttatgtttatttcacttgaacaaaagaaaaagcaactaataaaattgaaggaagagctgaactaccgaatatttttctttaactcaagaactttcagttacaggaagatttatctaatattaaaatgactaaattacaaaaagcataaaatgtttgaagccatttttaaagttgttttgaaatccatattagcactcagacttccccactccctaacttttgttaattgctgtaatggacatttgttgttttgatctacccaacatcctttcatcctactttggtaactgatattctttgggggaactgatctttccactttacatcatgttttgtggaaatttttcaactaaggaacctgccctatgctagctaagagttgagtacggtatgcaaactaaataagtgcaactctctcactgtaatttaacctccttaaatcaagtaaagaaaatgactgtggccaagtcacccctgctacctaggtccttgtaactgcccaggcacctctcccttctaaggcctatttggtcagcttgtcattttattctatcaggtcctccctaatgattccaataaattatttttgtttgtttttttaaaatgatccaaaccctggttttatggattgaaacagaagaatctatctgatataaaaatatttttactttgtgaaggtttgtaacattcttttctgtaattataattcctatatatcttaattatatacatgtgaatggatttaaacttaactttggtccaattataataatcttttatttgtacatgttgcttgcttagctagatttccttactgagtaacttttcttcaagaatgattcatgggtcctgtatttctagaactcttttatgttcaaaaatacccatgtgctgcctttgtactagaataatattttgactaggtttaatatttttaggtcaaaatttgtttccctaagaactgtacacatgttgcttcactgccttcttagatgcttctggtcaagatagaggaacagggaccatatttatcctccctcctgaaacaattgcaaaataagacaaaatatatgaaacaattgcaaaataaggcaaaatatatgaaacaacaggtctcgagatattggaaatcagtcaatgaaggatactgatccctgatcactgtcctaatgcaggatgtgggaaacagatgaggtcacctctgtgactgccccagcttactgcctgtagagagtttctaggctgcagttcagagagggagaaattgggtacagtgggacaggccttcaactcttgttttattgaatttatgaacttcttaaattcttctatggcaggagacatctatggggaggctttgtttgttttttgagacagggtctcactttgtcgcccaggctgaagtacaatggcctgatcttggctcactgtaacctctgcctccttgattcaagcaattctcttgcctcagccttctgagtagctggtattacaggcatgcaccaccacacccagctaatttttgtatttttagtagagacaggatttcaccacgttggccaggctggacttgaactcctgacctcaggtgatccacctgccttggcctaccaaaatgctgagattacaggcgtgatccactgcgcccaacttatggtgagttgtcttttgtcccctgagttatatatcctttcaggatgggttcttcatctggctcatgtcatatttcttttctacatttttccccattgtctttcgcctaatgatcagaacacttatctttctaatgcttaatcagggcagctgggtagagtctttctttttaccttaagatagtatagaagggctctctttgacaactttcttagatgaagtagactagtttggcttcttctccagtgtatagctggaggcctgggtggtgtcttccatctacttttgtgtagcctgatatgatctggtgtgagatgaggccctcgctgttaacctggtttctactctttattgttgcctaggaacttccattaaatccactgaattccatgaaggaggcaaagcatccaggaataagacacagcccccttcattgaattcatgtgaaatcctggaaaatccctcctgtgtccacggagagtccctggggacaatcaggagtttctgtgctcaagggtctccctggcatttccctgagctgcctgctcaatacctccgccaccacccttcaaactggccatattaacaagaattctggttttcttttctttatgtgacatctattcatgactacactgggcagatgagatagtagctatgcctttatataaaacttttaaattctttttttttgttttatttatttaatttttggagacagggtcttgttctgtcacccagactggagtgcactggtatgatcatagctcactgtaacctcagacttctgaggtcaagtgatcgtcctgcctcagccttctgagtagctaggactccaggtgtgcatcaccattcccagctaattttatttatttatttatttgtttgtttgtttgtttgtttttgtagagacagggtctcactatattgctcaagctggtcttgaactcctgggctcaaacaatcctcccaccttggcctcctaaagtcctgggatcacaagcatgagccaccatgcccaaccttttctagtttttaaattttcatacatatctattagatgtttatagtgtaaggttgaactccattctttgcttctctgttgctggtaaatttttgggtatatttttactaattttgcacattcttttacatattggtaaaggaacagtctgtgatctggatttattcagatccttattcagaattaccaattgttttattaatcattttatcttaaatgtgtctctacttactagtgatttgcagtatattccaagttagttgtaaaaacatttcacaatagactaatttcttgctttcctgtgaaattgtctcaaatttaaaaagtaaagttcttaatattgtaagtagctgccagaaataaaccaattctagcttcaagttcatacttcttacaatgagaattttaaatttctttattcttgggaaatagcagggccttgctgtttttaatagtgaattaactctgaattttttagtttctgtctctcagaaaagatggatttgtttggctttaaatattgagagagtttctagagacccacaggaaatgagaaatttgcacttttgtagcaatggcttttgaaagactagctaacatcctgaagactcagcagaagaaagatattaaactgactttgtcgttttgttgattattaaattaaatggaaaaacaaaatgtaacctttgagtccaatagactcatccccctaggctctctatcatcttcaaatcaatcagtaaaacacagtgtgcctccctgggggactgtggcagtcttaccttcatgtagtaacctaagacgctccataagaataaaaaatcagagctaaggaacagattccacataaccaaaaggctcacaaaaagcattttaaaatatagtgatcaaaaacactaatgtcgttaaaagaaaaagcagaaaataataaagtaatataatgtggtcttgcaaaaaacagtctgtgatcttacatttcaaaacatgtcttgcccgttcccggcacctacaaggccagatgagctacctgctccatccttcacattctcgctgcacgtcccattcaagctcttctgcaagtggccatgttaaaaatttataaaaatatccgagtctgcctggcacgctcagagattctcatgacaagttcttccctcactgagcacttccctgaccacccaaaataatcaccccctccatctacctacacacatgtgcacgtgcgcgcgcgcacacacacacacacacacacacacacacacacacatctctgagtctcacggtcctctaattactgatatccctttttaccatgggaaattccttgtctatctgtgtatttgtcagtggtctgtctctgccctaaaggaggaatcttacatcgattcgttctcaatccccagcacctagaaaagtatgtgacttaataagtgagtgtgtgcttacatgtttggattaaatggtttcacagttaattagagatgagaaccacttaattgtttcttaggcttgggtttcctgtcacacagaagccttcagaatatacagatgtctttttgccctagaagccaaacagagcagaagattgtaggccccagccggtggggctactcctggattgattccaaacacgatatttctttccaggcctgaaaatcgacagacactgtccaacacaatgtgatcggttagaacatccgacgcatcaccgatctgtagtaacagatcagactcctcatggagctgagacagttttctcttcctcattgctgttagaagcctgtctttatatttttccacttcacttgctttggtgaaaagcacagcaatatccttcggagaataaccattccgcaagagaaaacggcatttattcgctacatagatcagtatctcctccaagttcaagtcttcaataatctctaagttgcctgggacaccttgagcccatttaggttcatagagcatcaccagggacccaggggggaggttaggtggaggattttgtcgggcttcctgcattacttgttgtaggtaattagctattggacctgcattgcggaccactctgttgatctcttctcttggatactggtctgagggaggggggaggccactgcaactcaagtgataggtctgaaagtagtccagaaagatccagagaactcctgggccatcccttgctgtctgagtgatgaactttgctttcccataccagtccccatcttcagtacggaaattctgagcgtcatcaatgataatgtgctggatgtgttcaaagttgtttttcatgaaggttttccgggtcactggctggcagatgtttttcttgctgaaactcaccaacttcttcaggggctggttttcacagatgtagagaatgttagccggttcacagtgaaacacattcctgatcttctccatgatcctaagagccaagatagtcttccctgatccaggtaagccatgaacaaacaactctctggtcttgcgaaggttctttgaaagcaactcatactgtttatttgtcagtaggttcaaaacctcagagcccagctcttcacttaagaaggatttgaacccaagcaagactatcacgagggactgtaacagggcttccatgtgctggggggtcatgaagttataggattcagggtaaatttgtaaatacgaactgtaaacgctctgtgcttttctatcagaattcagcacacagaccaagggggtgatgcataacctcccagtgtagccgcctttgttcaccagcttctgcttcaaagaataggcaactatcatagaatagcccttgcaccccgcatcccacttgctgaagatggtgtagagaataggggtgttgttctgggaaattagaagagcatcacagatgactccctgcttctcttgcagacctaaatccacagcccagctttgagaaaaaatcaatattccttgagagaaagggcgcatttctgtatttattaagtctctgagtcctttatgttgtgagaagagttccttgtagaggctttctggagtatataccactctgtctgaaaatactggaaagtagcgtttctgctgctctttcagacattccgaattcttatgaatgcacacaggcttgctgcggggcgtggcagatgacaaactcaactggagaaccatctcaggacacctggaaaggtctgggtcagcttccatcatccaagcagtccattctcttgtgggcaattgtctcacacggttgtccttcacctgccaggaactaggcactttggcaaacaccgcacagcagaatttctccaccttgattgcacagacatatccacggagggcccccttatcatgcacttcaaggaagttaaggacatattttatctcaggcctctgtgtgcagaaatgatggacaggtagcttcttaatacagccatcaatagaagccctcaagctcgtaaggtctattttctctttttcacatccaatcacttgacaagtctcatcatgcacaccaaaaaatacatatcctccttcagtatttgcaaatgcagaaacacacttcggaagtctgtctttaacacagtgtgacacgtctgtcgagaacattacaaattcaacatgtgtggactcaggaaggttgagtttttccagatactgaagccgctttctatcaaataaagcagcagctgacacatttatgttaccttcatattgtacactaccctgagctgcctgtggacctaatgaattggaaacattaatattcgttggagtctgagtcctgcatttgaggaatgccagagcttcctgagaatccatgacatcggtggatgttctctctctgtggtacaaattggagcataaggtagcaagtggcacaccagcctctgtgttccatgatttcacaaaaatcaaaaagtggttttccttctgcatcttatctaaatggcttctgaaaattggaggcacatccaatcctactccatgacgttcataattgtagcctttgttctcaatctcagccttgattatgcccccaccagaattcagcagagcacatactgctcgcaggatgatttcattctgtttctcccgcaggcgagggtccatctcctgcctctgctgagtcccaagggtgacttttcctgcatctacaacacactcaggaaagtttgtatccacatcaatcctaagactcatcttctcagcacttggcctattcctatcctgaaatgttctcccgctgggttctcctcggcagcgcgtctccctccgggagcaggcaacggagcctcccaagtccagagcagag

SEQ ID NO: 9153 - RNA, 9044 nt, Homo sapiens
  source 1..9044: mol_type = other RNA
actttaacatggaagtgctttcccccttaaagtttgttaccaatctgagtaattttgtcaattgatacttctgctatcatgagtaatgtttccatatctttaggagctattttaaattctttttctgtattctaccacctgtcaaatcctttgctcatttttcctttgagaccttagaatttttctcttcgatttgtagaagctattttttgaaaataagaaattaactatttggctgtgatattcattgcaattctttttccagtgtgttgtttcttgaccttttatgctgtttttggtacagagataattttgtttaaaatagtcaatattttccttcctggtttctgattgagggccatacttagaccttccccatgctgagattattatttttttaagtgctacttcttcttcatgcacttccatgattccatatttttacttttaaaaacttggtcctcctggaatttattttggtatctagtctggcatatggcccaagcttaattttttttagctgggtgacagagttgttcatcatatattgaataatccatctttccccaattaacttgaatttaacatataaagttaacataacttaactttaacatatgctgttaatacatttcaacatgtattttaaatttatttttggccatttcatcttgttccattgaccctccacatatcagcaccacattgttttaattattgtagctttataagatgttttaatatttggtcatgctgactcactcaggtttcttcttttctagatttttcttggatattcttgcctcgtagtttccaataatttttttttttttgagacagggtctcactctggctgcccagactggagtgcagtgatgtgattttggctcactacagcctcgacctcccaaggcttgggtgattctcccacctcagcctcccgagtagctaggactataggtgcacaccaccacacccagctaatttcttgcattttaaatagagacgggatttcaccatgttgtccaggctggtctggaactcctggactcaggcaatccacctgcctcggcctctcaaagtgctgggattacaggagtgagccaccatgcttggccttcattaaattttaaaatcatttcaatgctattggggaaaacctgttggcatttttattgggattacactgaatttatagattaacagtgaaaattgatatatttataatttttaatcttcttatccaaaaacgtggtctgctttttatctgtttaagttcttttttgtgctctttagtttcattgtatagttttattgttgcagaacttatattttcttgttgcagttattcttaattattttatctttttgttggaattataatatggctttttctttcatcgtattttctaactacatgtagtctgacataataggcaattagaaaataatatgtatagacttaaccttatgtttcactaatttatttgttctcctttccttcttaaaaccactactttcttctcaattcattttttcttgttatagtacgttattcatatactcttgctaatagcccatccctatatgaatagtttttctgacttggaacaagtaggaagttttttaaaaatcacttatagtccatccctgtatgaagatgaatactataagtacattattcctacttgttccaagtcagaaaatctatttattttgccctcgactctgaatgatagtttggggagagaagtctaggtttgatgttgtttttccacagcagtttgaatatgctacctgtattctgcttacgtctacccttgctagtgaaatagttattgtcaaattcacacttctttttgtagattttccaaactttttcttttaggattaaaaaagaatctttgatgttctgaatcttgattgtaatgtgttatgcttgacctatatattctgccactattctggaaactcttttagtcaaaagaggtatggtggtggtgattttaccccccaagggacatttggcgatgtctggagacatttttggttgtcacaactgacaaccaaccctggggtaggggagggagggtggtggatttgctactggcgtctagggagtagggccaaggatgctgctaaacatcctacagtgcatagagaagcctctcacaataaatggttgtccagcccaaaaagccagcagtgccaatgctgacaaaccctgaggtatgggttttttagttctaggctttggtctggccaactgggggcaaaatgaatttggcttcagcctcagggcaacactttctggctgggagattctgtcctggctttgtgacaacggttgtcctggcctgtggtggtgccagcctcagtgtattaccgtggtttacctagattttccctacctgtaccaatgactcataggttttagttcatggagaggcgcttttcttggttgtgaggatggctatgcatatggcaatgttttgaaatatcttccccattatttctatgagtttgttttagtagagggcgatttcagcatgtgaccttcaaggtctttatgcaaaggggcaaagtcaataaaattaattctagcaatactgaaagagaaaaggaagcaataaatcactcataaactcatcaactagaaatattcaaggttaataatattccagaaagcttttaaaaatatatcagagaaaatataagaacagctagatagaattatgttaaatcgaaggatatgatacataatattttaaaattatttttatgtttatttcacttgaacaaaagaaaaagcaactaataaaattgaaggaagagctgaactaccgaatatttttctttaactcaagaactttcagttacaggaagatttatctaatattaaaatgactaaattacaaaaagcataaaatgtttgaagccatttttaaagttgttttgaaatccatattagcactcagacttccccactccctaacttttgttaattgctgtaatggacatttgttgttttgatctacccaacatcctttcatcctactttggtaactgatattctttgggggaactgatctttccactttacatcatgttttgtggaaatttttcaactaaggaacctgccctatgctagctaagagttgagtacggtatgcaaactaaataagtgcaactctctcactgtaatttaacctccttaaatcaagtaaagaaaatgactgtggccaagtcacccctgctacctaggtccttgtaactgcccaggcacctctcccttctaaggcctatttggtcagcttgtcattttattctatcaggtcctccctaatgattccaataaattatttttgtttgtttttttaaaatgatccaaaccctggttttatggattgaaacagaagaatctatctgatataaaaatatttttactttgtgaaggtttgtaacattcttttctgtaattataattcctatatatcttaattatatacatgtgaatggatttaaacttaactttggtccaattataataatcttttatttgtacatgttgcttgcttagctagatttccttactgagtaacttttcttcaagaatgattcatgggtcctgtatttctagaactcttttatgttcaaaaatacccatgtgctgcctttgtactagaataatattttgactaggtttaatatttttaggtcaaaatttgtttccctaagaactgtacacatgttgcttcactgccttcttagatgcttctggtcaagatagaggaacagggaccatatttatcctccctcctgaaacaattgcaaaataagacaaaatatatgaaacaattgcaaaataaggcaaaatatatgaaacaacaggtctcgagatattggaaatcagtcaatgaaggatactgatccctgatcactgtcctaatgcaggatgtgggaaacagatgaggtcacctctgtgactgccccagcttactgcctgtagagagtttctaggctgcagttcagagagggagaaattgggtacagtgggacaggccttcaactcttgttttattgaatttatgaacttcttaaattcttctatggcaggagacatctatggggaggctttgtttgttttttgagacagggtctcactttgtcgcccaggctgaagtacaatggcctgatcttggctcactgtaacctctgcctccttgattcaagcaattctcttgcctcagccttctgagtagctggtattacaggcatgcaccaccacacccagctaatttttgtatttttagtagagacaggatttcaccacgttggccaggctggacttgaactcctgacctcaggtgatccacctgccttggcctaccaaaatgctgagattacaggcgtgatccactgcgcccaacttatggtgagttgtcttttgtcccctgagttatatatcctttcaggatgggttcttcatctggctcatgtcatatttcttttctacatttttccccattgtctttcgcctaatgatcagaacacttatctttctaatgcttaatcagggcagctgggtagagtctttctttttaccttaagatagtatagaagggctctctttgacaactttcttagatgaagtagactagtttggcttcttctccagtgtatagctggaggcctgggtggtgtcttccatctacttttgtgtagcctgatatgatctggtgtgagatgaggccctcgctgttaacctggtttctactctttattgttgcctaggaacttccattaaatccactgaattccatgaaggaggcaaagcatccaggaataagacacagcccccttcattgaattcatgtgaaatcctggaaaatccctcctgtgtccacggagagtccctggggacaatcaggagtttctgtgctcaagggtctccctggcatttccctgagctgcctgctcaatacctccgccaccacccttcaaactggccatattaacaagaattctggttttcttttctttatgtgacatctattcatgactacactgggcagatgagatagtagctatgcctttatataaaacttttaaattctttttttttgttttatttatttaatttttggagacagggtcttgttctgtcacccagactggagtgcactggtatgatcatagctcactgtaacctcagacttctgaggtcaagtgatcgtcctgcctcagccttctgagtagctaggactccaggtgtgcatcaccattcccagctaattttatttatttatttatttgtttgtttgtttgtttgtttttgtagagacagggtctcactatattgctcaagctggtcttgaactcctgggctcaaacaatcctcccaccttggcctcctaaagtcctgggatcacaagcatgagccaccatgcccaaccttttctagtttttaaattttcatacatatctattagatgtttatagtgtaaggttgaactccattctttgcttctctgttgctggtaaatttttgggtatatttttactaattttgcacattcttttacatattggtaaaggaacagtctgtgatctggatttattcagatccttattcagaattaccaattgttttattaatcattttatcttaaatgtgtctctacttactagtgatttgcagtatattccaagttagttgtaaaaacatttcacaatagactaatttcttgctttcctgtgaaattgtctcaaatttaaaaagtaaagttcttaatattgtaagtagctgccagaaataaaccaattctagcttcaagttcatacttcttacaatgagaattttaaatttctttattcttgggaaatagcagggccttgctgtttttaatagtgaattaactctgaattttttagtttctgtctctcagaaaagatggatttgtttggctttaaatattgagagagtttctagagacccacaggaaatgagaaatttgcacttttgtagcaatggcttttgaaagactagctaacatcctgaagactcagcagaagaaagatattaaactgactttgtcgttttgttgattattaaattaaatggaaaaacaaaatgtaacctttgagtccaatagactcatccccctaggctctctatcatcttcaaatcaatcagtaaaacacagtgtgcctccctgggggactgtggcagtcttaccttcatgtagtaacctaagacgctccataagaataaaaaatcagagctaaggaacagattccacataaccaaaaggctcacaaaaagcattttaaaatatagtgatcaaaaacactaatgtcgttaaaagaaaaagcagaaaataataaagtaatataatgtggtcttgcaaaaaacagtctgtgatcttacatttcaaaacatgtcttgcccgttcccggcacctacaaggccagatgagctacctgctccatccttcacattctcgctgcacgtcccattcaagctcttctgcaagtggccatgttaaaaatttataaaaatatccgagtctgcctggcacgctcagagattctcatgacaagttcttccctcactgagcacttccctgaccacccaaaataatcaccccctccatctacctacacacatgtgcacgtgcgcgcgcgcacacacacacacacacacacacacacacacacacatctctgagtctcacggtcctctaattactgatatccctttttaccatgggaaattccttgtctatctgtgtatttgtcagtggtctgtctctgccctaaaggaggaatcttacatcgattcgttctcaatccccagcacctagaaaagtatgtgacttaataagtgagtgtgtgcttacatgtttggattaaatggtttcacagttaattagagatgagaaccacttaattgtttcttaggcttgggtttcctgtcacacagaagccttcagaatatacagatgtctttttgccctagaagccaaacagagcagaagattgtaggccccagccggtggggctactcctggattgattccaaacacgatatttctttccaggcctgaaaatcgacagacactgtccaacacaatgtgatcggttagaacatccgacgcatcaccgatctgtagtaacagatcagactcctcatggagctgagacagttttctcttcctcattgctgttagaagcctgtctttatatttttccacttcacttgctttggtgaaaagcacagcaatatccttcggagaataaccattccgcaagagaaaacggcatttattcgctacatagatcagtatctcctccaagttcaagtcttcaataatctctaagttgcctgggacaccttgagcccatttaggttcatagagcatcaccagggacccaggggggaggttaggtggaggattttgtcgggcttcctgcattacttgttgtaggtaattagctattggacctgcattgcggaccactctgttgatctcttctcttggatactggtctgagggaggggggaggccactgcaactcaagtgataggtctgaaagtagtccagaaagatccagagaactcctgggccatcccttgctgtctgagtgatgaactttgctttcccataccagtccccatcttcagtacggaaattctgagcgtcatcaatgataatgtgctggatgtgttcaaagttgtttttcatgaaggttttccgggtcactggctggcagatgtttttcttgctgaaactggaaagtagcgtttctgctgctctttcagacattccgaattcttatgaatgcacacaggcttgctgcggggcgtggcagatgacaaactcaactggagaaccatctcaggacacctggaaaggtctgggtcagcttccatcatccaagcagtccattctcttgtgggcaattgtctcacacggttgtccttcacctgccaggaactaggcactttggcaaacaccgcacagcagaatttctccaccttgattgcacagacatatccacggagggcccccttatcatgcacttcaaggaagttaaggacatattttatctcaggcctctgtgtgcagaaatgatggacaggtagcttcttaatacagccatcaatagaagccctcaagctcgtaaggtctattttctctttttcacatccaatcacttgacaagtctcatcatgcacaccaaaaaatacatatcctccttcagtatttgcaaatgcagaaacacacttcggaagtctgtctttaacacagtgtgacacgtctgtcgagaacattacaaattcaacatgtgtggactcaggaaggttgagtttttccagatactgaagccgctttctatcaaataaagcagcagctgacacatttatgttaccttcatattgtacactaccctgagctgcctgtggacctaatgaattggaaacattaatattcgttggagtctgagtcctgcatttgaggaatgccagagcttcctgagaatccatgacatcggtggatgttctctctctgtggtacaaattggagcataaggtagcaagtggcacaccagcctctgtgttccatgatttcacaaaaatcaaaaagtggttttccttctgcatcttatctaaatggcttctgaaaattggaggcacatccaatcctactccatgacgttcataattgtagcctttgttctcaatctcagccttgattatgcccccaccagaattcagcagagcacatactgctcgcaggatgatttcattctgtttctcccgcaggcgagggtccatctcctgcctctgctgagtcccaagggtgacttttcctgcatctacaacacactcaggaaagtttgtatccacatcaatcctaagactcatcttctcagcacttggcctattcctatcctgaaatgttctcccgctgggttctcctcggcagcgcgtctccctccgggagcaggcaacggagcctcccaagtccagagcagag

SEQ ID NO: 9154 - RNA, 3171 nt, Homo sapiens
  source 1..3171: mol_type = other RNA
actttaacatggaggcacttgctccacagaggagcatgatccttctgaacagggctgctgattgttcctttcatttcttcttgtgaccttgagctcccttaaaaaaaaaatttcagtggagaatcacagctggtaatgtactgcgagttcttgaagctacacaaggtatagtctggctaagttacatgtggtttccatattagcttgtttggcagggtgacctactgcaaagcaggctcagttaccccaccagtcaaccccctgggagttataatttcctccatatccatcactgttgtaaaagcctccatagccacctccaccaaatcctctgctgctaccgtggccacctccgccactgcggctgctgcttgcgcggctgctgctgaagctggaactgctggcaccgctactttgtcggtagtctctggcaccaaaccctccactaaatctgctactcttagaacgtccacgactgctacccttgtagtggtgttcataagccatgttttctaaccaagacggcacttcttgtttagcttcaacaagaagatccaacaaatccttagtaatatttatgttcctctcgttaaagaatgaggttgccaggccaaggtttcctacacgtcccgtacgaccaatacgatgtacatattcttcaatatcacttggcaagtcaaaattgataacatgtttcacatttgaaatgtccagtcctcttgctgctactgctgtagccactaaaattgggctttttcctgagcggaactggtgaagggcctcttctctatccctctgagaacggtctccatggatgctggtacatgcgtatccttcatggtataagaaatcctccagagaatctgcaccctttttggtctccacaaacactaaggtcagtgaatccttgcctgttgcatttaggaggtcaagcagaaatgaccgtttgtctgattcttccacccaaactactttctgtgtgatgttttcagaggtagagccaactcttcctacagccaagaagatatattcatctaagaaatcacgagccagcatctgtatttccttaggaaaagtagcactaaacatcatagtgtggcggacaccctttggaggcatagtatcttgttcgactattctacgaatctgaggctcaaaccccatatccaacatccgatcagcttcatctaacaccaagtatttgcaaaagtctaatccaatctttcctctttccatcatatccactagacgtcctggagtggctactaacaaatggcatccacgttccaagtctcgaatctgctgaccaatatcggcaccaccataaaccacgcaaggacgaactctagatcggtatgaaaattttctggcttcctcgtagatctgtactgccaactctctcgttggtgctaataccaaggagattgggtattgtttgcggcgcccataccttccattttccttcatggccctcaaagcctcgcctggaccatctgaataaatctgactcaagatgggcaacagaaatgctgcagtttttccagaccctgtttgggcacaagccatcaagtctcttttctctttgataataggaatagcatgcttttgcactggagttgggcgagtataacgagtaagctcaatgtttcccatgataatttctcccatctcaacatcactgaaactttcaatatgtggaggacagttgttgcctgttgcctcaactggaatgtcatcgtatttctcaaaattaatcccagtgttgcctccagaaaagagttcctgttccaagcgttcacttggtgggagtggttttgaccaatcatcttcatctgatttgtcacaccagcgactgtttccaccacgttcaaatttgccaaagccacttctgtcaccacggctgccaatgccatcgtaatcactccgtccacgatcatcaaaccttccccttgatccacttccacgatcactgaagaagctagacttccctcttgaatcactacgagatccaaaactgctatacgcatccttatctttgctagaactccaccctgaactgtctttatcgtagaaacctttagtagcttctcggttccttaaatgaggaggaatatagcgccctttgctggctgtacttcctccactctgattatctgaagagttcaggtctaggccagcaaactgctggtccagcccgagcgcattttccactgccacatgactcatccctgaagagtaccgagaactcggagtcttccgctgctaagcgagtgtttgttccaccgcgaaggccctctcacgggagaactgcggctctggagcgcaccgcgcggccacggatctaatatacccgctggaaagccggctacgtcagcacgtacaacgtgtgccctccctctcacaccgcaattccctgtcgcggcgacttctgcccggctactgcgcgctccctcaggtctaagctcaagggatttcctacttagtcctgtcgcccctagcagtcctgccttggagcttagggtgcgaaatgctgtcccagttctctcgagctacacttcccgtgctctccgctaaaaccctagtctcagcctcggagttctcgagatctcgcgagaacttgcgtctcccgctttccaccggctaagacgcctgaaaatgttaacctaggcctcttcgcccccctttccaaccttacgcattcgctcccctttccaactctatgcactcagctttcgtttttcgttttttttgtttttgttttttttttcctaacactggccttcactcttcttcctctctcagttcccgggcttggagatgtggtgggatttctccggtctaatctgccctcgctcttccgcgggtagcctccccttagtgggagctaggcagattcccgaaactgagagggcggcaggccacgtgaccgtaggtgtcgcgtgcggtggccattttgtgaagcaggaaacggtggcttgaatatagagtgctccggacgggggaggggaggggaagaggaggagagaacagagggaaggggaggagagggagggaaaagaggggagcggagtaaggggaaaggaggagggaggagggtaggatggtgaccggggcgggagtcggggggaaatggaggggagccggcggcgcgcgcaggtggccggacacctt

SEQ ID NO: 9155 - RNA, 23 nt, Homo sapiens
  source 1..23: mol_type = other RNA
agaaagggtggcaatacctcttc

SEQ ID NO: 9156 - RNA, 590 nt, Homo sapiens
  source 1..590: mol_type = other RNA
agaaaggtggaggggttgtcagaatctgtgttctcatgggaatgcctggggatcctcttgcagttgtgtctttgtgtaatgagagttactcaggcagcactcttgaggttcccctgaggggctccttccgagccctggagtcatgctgcccctcctgagcacctcggctcttgaggctccaggttcctgttgcacctggcaacccgggagcagcttagctgggtgattctggctcagaatctctcatgaagttgtggttaaaatgtcagccagggctgcaggcatccgaaggcttgactggggctggagggtctggctccaagatgccactcacatggctgctggcaggaggcctcattgctttaccatgcagatctctccaatgagctgcctgagtgtgctcatgacatagaagctggtttgtcccagagctggctccgggagaccaggtttcctcgtctggggagcgcagcagtctcatagctgccgtgagagggttcgcgacagaatcaccgcgaagggcgggaggacccggatcgtcgggagaggtgggctgcgtgcagccactgcgcggggacccggatgcacgc

SEQ ID NO: 9157 - RNA, 695 nt, Homo sapiens
  source 1..695: mol_type = other RNA
agaaaggtggaggggttgtcagaatctgtgttctcatgggaatgcctggggatcctcttgcagttgtgtctttgtgtaatgagagttactcaggcagcactcttgaggttcccctgaggggctccttccgagccctggagtcatgctgcccctcctgagcacctcggctcttgaggctccaggttcctgttgcaccttggttcttcagaatatgtagtgggggtggtagagatacacgtagggatatctggtaggtgtgacaacattcttccagtctcagccacttccagaagctgcccaagtccttgagactaggtgatggtcgggtggaggaggaagtggttagggaagcagagacccagatggctgcctcagtcctaggtaggatgagggcctaggggtagagtctccctggagcaatctgaggactcactggataatccaccctctgtcttcctccagggacctgggccctctggagcctcttcctggagcctcgttgtggatgagagccaccctggcctctgccccgaccctggacatgtctagcagggctggcaccagctgccccccagcaacccatgagccgactccagccgccgggggcctgtgttgcaagctgggcctcttactgctctccctgggcttggcctctcctccccagttggctcggctggtctggaaacaatgactgt

SEQ ID NO: 9158 - RNA, 573 nt, Homo sapiens
  source 1..573: mol_type = other RNA
agaaaggtggaggggttgtcagaatctgtgttctcatgggaatgcctggggatcctcttgcagttgtgtctttgtgtaatgagagttactcaggcagcactcttgaggttcccctgaggggctccttccgagccctggagtcatgctgcccctcctgagcacctcggctcttgaggctccaggttcctgttgcaccttggttcttcagaatatgtagtgggggtggtagagatacacgtagggatatctggtaggtgtgacaacattcttccagtctcagccacttccagaagctgcccaagtccttgagatggataatccaccctctgtcttcctccagggacctgggccctctggagcctcttcctggagcctcgttgtggatgagagccaccctggcctctgccccgaccctggacatgtctagcagggctggcaccagctgccccccagcaacccatgagccgactccagccgccgggggcctgtgttgcaagctgggcctcttactgctctccctgggcttggcctctcctccccagttggctcggctggtctggaaacaatgactgt

SEQ ID NO: 9159 - RNA, 903 nt, Homo sapiens
  source 1..903: mol_type = other RNA
agaagaaggcggtcggtctgcgggagccaggccgcagagccatccgccttctgtccatgtcttctttatcttcctcgccataataattagtggtgtggacccccccacacacactttttttcggatttacttgtatggaaccattcggacaaacgtgtgaacacaatgtcacaataggtgaatccagacaatgagctcacagacgaataaacgcagaggcacacacatatactccggaaaataagcagggcgccttttcactaacaaggcgcaattgtaccctgagctgccctccagaccgttcccctccctcagagccaaactcccgcagcgaatctctcagcaagctacgaaatgggatcacagggtcgcgtctacgcgggctccaggcccgaaataatttctaactccaaagcaagtggattttattaggcctccagaagccgaataagggagtagtggcgcaatgcgtagaaactacctccggaagctctttttgaatctcggttccagcacccgcaacgcagagcgcgaacctgaggctccatctttcgggttttactccggctggctagcgcttccgggaaccctgcgaggccgccgccagccgagaatccgccccgccttccctgcaggcgatccctactccaaatagtagttcccgggccggaagctggaaagccctcgaagcaggaaaaagcctcatccaggccccccagttctcgggagcagctccagctttccttccccaacctagagcaaacttctcttccctgcagctcccctcccccccttcattaaagttatattgaaggtgctaagtgctgcactctaattgggtttccttcaggggagaccctgtgccccccggccccaacccgtcctgtctaatagaaatccccg

SEQ ID NO: 9160 - RNA, 270 nt, Homo sapiens
  source 1..270: mol_type = other RNA
agaagaaggcggtcggtctgcgggagccaggccgcagagccatccgccttctgtccatgtcttctttatcttcctcgccataataattagtggtgtggacccccccacacacactttttttcggatttacttgtatggaaccgtaaacttgcaataaagcccggaggcgactgctgcggagggggcaaaagaaggtttcgttgtttttgaaatttataccattctcaccctcccgaacagtcgctctccagggaagaggggagaaagctc

SEQ ID NO: 9161 - RNA, 158 nt, Homo sapiens
  source 1..158: mol_type = other RNA
agaagaaggcggtcggtctgcgggagccaggccgcagagccatccgccttctgtccatgtcttctttatcttcctcgccataataattagtggtgtggacccccccacacacactttttttcggatttacttgtatggaacctatattcgcctgcaga

SEQ ID NO: 9162 - RNA, 221 nt, Homo sapiens
  source 1..221: mol_type = other RNA
agaagaaggcggtcggtctgcgggagccaggccgcagagccatccgccttctgtccatgtcttctttatcttcctcgccataataattagtggtgtggacccccccacacacactttttttcggatttacttgtatggaacctccggaagctctttttgaatctcggttccagcacccgcaacgcagagcgcgaacctgaggctccatctttcgggtttta

SEQ ID NO: 9163 - RNA, 213 nt, Homo sapiens
  source 1..213: mol_type = other RNA
agaagaaggcggtcggtctgcgggagccaggccgcagagccatccgccttctgtccatgtcttctttatcttcctcgccataataattagtggtgtggacccccccacacacactttttttcggatttacttgtatggaacctctccctgcaaggcccttcagacactaacaagcacctgcttccatccggagtcacccagctgagatcacac

SEQ ID NO: 9164 - RNA, 3254 nt, Homo sapiens
  source 1..3254: mol_type = other RNA
agaagattgcagagtaagttccccaacagtcagaatttgtccctgaagaaggttaaaccttaaacacctgcttcaaaaaaccaaaacaaaataacccgaaaaaaaaacaaaaacaaaaaacaaaaacaaaaacaaaaaggaaaaaaagaaagcaaagaaaaggaaagaaaaaagaagaaaaccaaaagaaactctaagcctaagggcttaaaaattacaggcatagccttttctctattttctatatttatatgaaaataattcatgcttcatgctaaatacattatttaccttacaagaactttgttacttttgaataaaaaaagtttgtttttgtgatttttttctctttttcttttttttcttcaaaggaatccatgcattgtggatcagaaatttctgctggctatactggctgaatgtggaaatcactgatttttgcaaagataaatcctgatattaattgcaaactccattttgagggcagtataggagttattttattttttgccatgttttactttttttttttgtccatcagtgtacctttaatcttaaaaatacaccacaatactaatggcaggttccgtagctttctagtttttttttttttttcacttggatcaaatagttttgatagacagaaaaagatctgtaccattatttcctttccttaacagctattgtaatttcctggacttggttgcttttcacttgggcagttaagaagacacagcttgttttccccatcagttttctctctctctccttcgtgtgtgtgtgtgtgtgtgtgtgtgtgtgtgtgtgtgtgtgcgtgcgtgcacagggccaatcttcaggcttatggcttttggaacattttcttaatttaatagagaacagaattcaatgattagcaacatcactaaaaatttaccccatttcttctccatgagtcactgacacccgatgcgcatgaacagtccaacgtccacctcgtaagatgtcatcgggcttcagggttcagaagcatcgaggactggtggccggccctctgtgctcgccgtgtgacaattccagtggctttcctggcaccatcagatgcctggtgccacaagcttgggtctgctcctagggggacgaggggttcctcctcctcctcaattgctttatgtgccttcactcagtgaacccaatgggatggacaacctgactttttaaacctaagggttgggcctgaacgatgattactttgcccacgtgccttctaggtgccgaatgtgtgttcctgtgatattgacgttgacatccctgcggattcagccacaggtttctgacaagctggaggaagcaatggtaattttggctttttcggttttgtcttcagataatgaaaagcttttgtaaaacagctgagtgtcaatatgagttctatggcttcaatctcctttaaaaataaaattcttaagggtccaaaacaaagaagagggggcaaattaaaacaaaataaaaggaaaagaaaagaaagaaaaccaaaccaaaaacaagaaaaaagaaaaaaaattgctgatattgccacaaatcattagaaatctcctgacatgctgaaaccaaatggtcgtaagttcaaaacaaatcagtgacttgtttttaattttttgtggtttccttttgctctttctgcccctttgccgtccgattggtgatgttattcaaacaggaccggatccctgctaagtgcaggagggaccctgccgcttctttcatctcctcatcatcgctctcggggggcttttcggtgcgtctctttttgaggggcagtgtgtcgctggggaccttcctggccttggcgaagtgctggcgcttcttgtgctgggatgcgtacccgctgtcccccagagaatccttgggctccttctggctgtgcttcctgtcgtcctcttccgtgtcgctggggctctcgtggctccggaagctcccctcgctgccctcgctgccctcctggctccccttggtggcaaactcatagtggtcgtcggctgaggaggaggaggaggagatggagtcgctggtgggcgaggtgctccgggcgttggaggacttggcactgctgtagttgtgatcctccttggggtctccgctgaccactggggagccacaagatggctcactctcagtccgcatccggcagctggtgatgccattcctcatggccgctgtcaccccaatgggagtgattggcagcggccgcacgccaggaaacagccctcggctcaggacccgcgctccattttggatcactcctggaggaaaacctgcttgtatctcagggggagtattcaaaagcatcatggcactggcagcatcaatgtcaggatcttggagaagggctccatttctcttgaagaaggtactgcccggccagatgggtggacctgatgtgctttgatatgcctgaggacaggtgggaggtgtattgaacacgtgtgggtgtgggtgataaggtgtctttttcaaagcctgaattagattttgtctatactctgggtctatgcaccacaacgaccctttcccaatactctgactcctctctttgtccactttcttaaaacacttattcaatgataaattgtgtctcactgagtttttccacccagtaggtgcatttgcaaaatacggaaaatgttccaagatccagttgtagatatccttcactggcaggcgcttggttggagagtcctcgatggccataaatatgaggcagctgaaggagtaggggggtttgcagttggggttctgcctggcatcgtagggcatgtcagagtgggcaggggatgggggggtgtcatcgtccaggtcctggacggggctgacactcctgaggaccgactccccaaagctcttcagcaagttcttgctctcgtgcagccagttcaggttggtcagctcttcatcttccatggccccctcttctaatcggatgtcaggcagagaaaagtcgaggtcatcgtcttcctgaagggccttggagaaaccgctgcccccgtaacactgactcagtccactggagacactaattcctgagctttctggcttcttactgggaggcatgactggacccatttacgtgaaggctccttcgatcgcctgcccccccgctgcttctcgcggccgcattggggggctgcggcgacgctggactcgcgggtggccccgccgccgggtcgcgccgtctcccggccgagctgcagcagatcgcggccggaaccccggct

SEQ ID NO: 9165 - RNA, 3413 nt, Homo sapiens
  source 1..3413: mol_type = other RNA
agaagattgcagagtaagttccccaacagtcagaatttgtccctgaagaaggttaaaccttaaacacctgcttcaaaaaaccaaaacaaaataacccgaaaaaaaaacaaaaacaaaaaacaaaaacaaaaacaaaaaggaaaaaaagaaagcaaagaaaaggaaagaaaaaagaagaaaaccaaaagaaactctaagcctaagggcttaaaaattacaggcatagccttttctctattttctatatttatatgaaaataattcatgcttcatgctaaatacattatttaccttacaagaactttgttacttttgaataaaaaaagtttgtttttgtgatttttttctctttttcttttttttcttcaaaggaatccatgcattgtggatcagaaatttctgctggctatactggctgaatgtggaaatcactgatttttgcaaagataaatcctgatattaattgcaaactccattttgagggcagtataggagttattttattttttgccatgttttactttttttttttgtccatcagtgtacctttaatcttaaaaatacaccacaatactaatggcaggttccgtagctttctagtttttttttttttttcacttggatcaaatagttttgatagacagaaaaagatctgtaccattatttcctttccttaacagctattgtaatttcctggacttggttgcttttcacttgggcagttaagaagacacagcttgttttccccatcagttttctctctctctccttcgtgtgtgtgtgtgtgtgtgtgtgtgtgtgtgtgtgtgtgtgcgtgcgtgcacagggccaatcttcaggcttatggcttttggaacattttcttaatttaatagagaacagaattcaatgattagcaacatcactaaaaatttaccccatttcttctccatgagtcactgacacccgatgcgcatgaacagtccaacgtccacctcgtaagatgtcatcgggcttcagggttcagaagcatcgaggactggtggccggccctctgtgctcgccgtgtgacaattccagtggctttcctggcaccatcagatgcctggtgccacaagcttgggtctgctcctagggggacgaggggttcctcctcctcctcaattgctttatgtgccttcactcagtgaacccaatgggatggacaacctgactttttaaacctaagggttgggcctgaacgatgattactttgcccacgtgccttctaggtgccgaatgtgtgttcctgtgatattgacgttgacatccctgcggattcagccacaggtttctgacaagctggaggaagcaatggtaattttggctttttcggttttgtcttcagataatgaaaagcttttgtaaaacagctgagtgtcaatatgagttctatggcttcaatctcctttaaaaataaaattcttaagggtccaaaacaaagaagagggggcaaattaaaacaaaataaaaggaaaagaaaagaaagaaaaccaaaccaaaaacaagaaaaaagaaaaaaaattgctgatattgccacaaatcattagaaatctcctgacatgctgaaaccaaatggtcgtaagttcaaaacaaatcagtgacttgtttttaattttttgtggtttccttttgctctttctgcccctttgccgtccgattggtgatgttattcaaacaggaccggatccctgctaagtgcaggagggaccctgccgcttctttcatctcctcatcatcgctctcggggggcttttcggtgcgtctctttttgaggggcagtgtgtcgctggggaccttcctggccttggcgaagtgctggcgcttcttgtgctgggatgcgtacccgctgtcccccagagaatccttgggctccttctggctgtgcttcctgtcgtcctcttccgtgtcgctggggctctcgtggctccggaagctcccctcgctgccctcgctgccctcctggctccccttggtggcaaactcatagtggtcgtcggctgaggaggaggaggaggagatggagtcgctggtgggcgaggtgctccgggcgttggaggacttggcactgctgtagttgtgatcctccttggggtctccgctgaccactggggagccacaagatggctcactctcagtccgcatccggcagctggtgatgccattcctcatggccgctgtcaccccaatgggagtgattggcagcggccgcacgccaggaaacagccctcggctcaggacccgcgctccattttggatcactcctggaggaacttggagaagggctccatttctcttgaagaaggtactgcccggccagatgggtggacctgatgtgctttgatatgcctgaggacaggtgggaggtgtattgaacacgtgtgggtgtgggtgataaggtgtctttttcaaagcctgaattagattttgtctatactctgggtctatgcaccacaacgaccctttcccaatactctgactcctctctttgtccactttcttaaaacacttattcaatgataaattgtgtctcactgagtttttccacccagtaggtgcatttgcaaaatacggaaaatgttccaagatccagttgtagatatccttcactggcaggcgcttggttggagagtcctcgatggccataaatatgaggcagctgaaggagtaggggggtttgcagttggggttctgcctggcatcgtagggcatgtcagagtgggcaggggatgggggggtgtcatcgtccaggtcctggacggggctgacactcctgaggaccgactccccaaagctcttcagcaagttcttgctctcgtgcagccagttcaggttggtcagctcttcatcttccatggccccctcttctaatcggatgtcaggcagagaaaagtcgaggtcatcgtcttcctgaagggccttggagaaaccgctgcccccgtaacactgactcagtccactggagacactaattcctgagctttctggcttcttactgggaggcatgactggacccatttacgtgaaggctcctggccggagcggggcacgggggtgcgggggcgccgctgcccttcagcaggagccgacaaactttcgcgggcgcccggcgggcatcgctcggtggccccgctaaggacgcgcgggcgcggcgcggcgagcccggggcggcgggcggcggggggcggccgcgggcgcgggcggcaggggcgcgggggtcgcggcgcggcatgggacctgcggcgtccgccgggcgcgccgcgcgtcctcccgccggccccgccgctctccccgccccgtcccgcctcccgctcgcctccgccgcggcgcgtcgggccggggcgcgccgagcggcgagaaattgtttccactgcaaacaaaaaaaggcgacacat

SEQ ID NO: 9166 - RNA, 102 nt, Homo sapiens
  source 1..102: mol_type = other RNA
agaagggaagatggtgacaaggaattgctaagcagcaggtcacatgggtcacccagcgtggaccggcctgaacacagcttccatgtccccactcttgccaat

SEQ ID NO: 9167 - RNA, 1841 nt, Homo sapiens
  source 1..1841: mol_type = other RNA
agaagggaagatggtgacacatgacaggagcaacaagaagggcagatggggacacaggtgcaggaggagaaacaggggtctacggggtacagtcaggcaaggggtaagatggagatgcagacacacaaacccaaggaacggaaaatggaaaggcagggagagggaggaagaaagagaggaacaggagagagagggagagagagagagaggaatgcagacaggaggaaaaatgaagacacaaaaaggaggcaaggaaatggataaaaccgagggggaatgggctgaagggaagggggagaccccggcagaaatggagaaatgggggcgcagacagacgggaagagtgaggttggagtgcctttcccgcgctcatcttccgtccccactccacgcccagcaaatccaaacaccgcggcctctggtgtcccggtctccactttcccctgaggggcatgggcgtctcctcctccgcccagccggggcgctgagcggcggtaacagcggcggtggctttgtggtcccggggggtccgagtgtgtgtcaggggctggggcgggggatgggcgcggcccctgggtatccctagcggtccaggttcatagtccagtgcttggttccggccgcgcagctgtccctggcggccgaggaggcggcgggcgcgcccccgctcggtgggcccccgccgctggcggcggcctcgccctcgttcttgaggtcttgaaagacctgcgtgaagaagtgggggtcggcgttgagccgcagcatctgcgggctgagccgctggatgaggcgcaggcagcgctgccagaagcgctccttgtcgggctccacgaggaagggcttgagtgggtaggagatctcgttgcccatgtaggagtaggcgaggtagaggcaggtgaggaaggcggcctgcagctcggcggccgacgccagctcgtccccacgcagcgactcgcggcacagcaggtacacgaacaccaggtttgcaggcgtaatgaaggcctggtcttgccagccctgcagcagcagcgagcggtccacaccgcggaaccagcccaccagctcgcccgggctcagctccttgaggcgatagcagcgtcggcacacgaagtcgcccagacagcgcagcagctcgccggtggacgcctgcacgatgacccgccgcggcgagccgccaggcaccggcggcgccacctgcggggctgggggaggcggcggcggaggctttcccccgcccgagcccggcggctgagcggccgcgctgccccccgacggtggctcgcaggtggcggcagccgcgggcacggtgggcactggcaccgccaggggcttggcggtgccgccgccgtcggggggatcccggcccttgcggagaaggttctcgcggttgcgttgctggaccagggggtcggggcccgtggatgccggcttgggtgtcaccttcttgctgcctttcttcttcttggcggacgcggccaccaggcgcttccaggtgagcgccgagatgagcacggacggccgcttgagtcggctctcgcctttgccgcccttgcccactggcggcgccccgtagccccccagcgcctcgtcccccgcgggcggcgccttcttcttctcctcgggcagcccgccgggcctccggcccttggccgaggaggcaggcgaaagagacagcactgtgcccatcctgcagagcggggccggcgcccaggccccagcgggagccgcgggcggcgccgctgctactgcagccccgggggacccggcggtggggggcctagccccggcccgggcgcgcggactggcgggggaaggtggctgctaggcggctccgctgctct

SEQ ID NO: 9168 - RNA, 2175 nt, Homo sapiens
  source 1..2175: mol_type = other RNA
agaagggaagatggtgaccacataggagggacagcggcctttccaacaggggacccttgccagccatggtgagtagatggaatctgtgcccatcctctgcaagcccctagcaaacgtgtgaccaggaaagagtctgagatcatgtcacatttcctgagatgagcacgtaggtagaagctccttcctttaagctttagttcttactggggatggaaattccatccaacaaatgttgatatagcttgcttccttctaaggggatttccagcaggtggaaattgaattgtgagggaacaagtaaatcttcccagagtgtctgaagtcacatcgcagccttagcttttagccggggctttgtccctcccttctaggacagtctccatgacctcagctgaaaatgggacaaagtggggacctgtgagtccttacacttgcagttttcacagggctgctcagctttgagcttggccactcccatcctcagggtgtcccaatctgagatccaggaaatcaggaagactaagaggctggtgtcatggcccagggcagagcctacctgaatcatagctgaaccagcaaatgggggtgggggaagatgaaggctgagttctccagttcccttcattggcttccaggtgtgcaggtggcttgggattgaggactcagatcttctcaggccccgagggcatcgatgccagcagggctgagcaccagtgcctgaaggatgtcggagagggagaccacgcccaagagatgctgggtctcgtccactagcaccagcctgtgtacctgctcccgagcaatcctgtcgatcacttcccccaagctctcgtggggctggcaggaaaggactccctccagacatagtgtcctctgcctcagggcttctcccacactcatgtccaggtggttgtaggtttgctgggcagccaggtgaatcacatcaaagcgggaatagaggcccacgacctgaccacattcgttgaccacaggcagtgcagacacacgccggtccacaaagatgtccagtgcagtcaggatgggtgctgtctccagcaccacagccaagtctcggaatgtgccgatgcccaaatcttggatagtgcggtagaggaaggagggccggggcagcagggaaccaaagatgtgcaggaacttgagcaggcgtttgtgtgtgaggatgtggagtacgttgcctgacaccgggtcaagaacaggcaggcgatggatccggttcttgatgagggtgtagacagcttcaaacaggctatcattaggagagatggagaccagaggcttgaagcagccttgcaggtagatctccctccaggtctcaatcttatgttgttcaatctcatagatctggaccaggggggacctgtagtagcgatgcagcaccaggatgaagtcagtgatggtcagcatccccacaaagctctgcttcttgctgtcccatagaggggctgcccgcacaccgttggccaccagagcaaagaaggccttcttgatctccagcatggtgtcgaagatgactagcttggagctagttgccatggcatcgtagcaggtgtgctcctgcatgaagcgcatgtagatctgggcgccgggtttccgcagttcgtcatcccagcccagcttgggaaatggggcctgcggggacaggcacagggcaggcctctcttccagcaggccttctagctcacactcccaggcctctgtggctgggaactccgtggccagctccacatcatctgtgctggagcctgcagctgaggctgtacagtcagaggggaggcagtcccaccctgttggtggagtgcccaccccggcaggatcagcttgagccaagggtgtggtcttggggaatgtggcctccagcccggtggactcagcagctggcctggaccggggaccttccccctgacctggtggctccccttcctccaccgacttctgccttgtccatctcaaggctttggccctccgtttcccacggattctttctgagctgctggtcacagctggtgatggccatgagctgctgttttcttgctctaggaagctcatctcttgatgctcagaacccccaaggctgctccaggaaggggtcctgcgcagtgcgtgctccagcccgggctccatgtggccagccccagaccaactgagagcaagtgt

SEQ ID NO: 9169 - RNA, 892 nt, Homo sapiens
  source 1..892: mol_type = other RNA
agaagtaattgcggttttgccattacttttaattgcaaaaaccacaattacttttgcaccaacctataattgctccaaccacaccgaactctttgcagatcagtttgttcaaaaccatcttaatcaccgtctccaccctccccttccagcctcatctcctactatattccagcccaccccttgttcatctctttgatgacctaaaaattcagtcttcattcttttctctccaaacttttgctcaagtttcccccaaatatttagaatagctttaagttcatcttttctggaacattttccttaataaatccacctcattgcacacagctgcctagatgtagcctcagccccattcctctctctctttctcaatcccacttttgtgattattgtatgtatctgcatctgttttctgtttagcttccaatatgagtcctagagaacatctcatctccatcatatgtccaggaaaagcttgttgattgactgaatactccaggtgccacaaaggaaagttctttagggatcatagttgttgctgggttttttgttttttgttttaattaaaaaaaaaaaaaaactcttgagtaaaggaaggaatacgatccatctgatctttctgagacttccaggctctgtcaacaactatttggaaataaattcttaggcaattagatcatggtatcttctttcagacagcatagggaaatgaatataaactctggggaaagccaaccaccatgtctgtgatgaggccactcaagcagcctatggcaagcagtccacatggcaaggaacagaagccccttgccaacagccagaatgaacttcctaggcttgtgtgggagttgccttgagaggaggttctccagccccagtcaagtcttcagat

SEQ ID NO: 9170 - RNA, 1097 nt, Homo sapiens
  source 1..1097: mol_type = other RNA
agaagtggctaataatattgaaaaccacttctgctgcagccacctgtagaggcttccccacccagagcatcatcctgtgcgtctcccaggggctccccagcctgtgatgagtgggtgacccccatctcccctggggcagctgcagaggcctctgcccaagcagcttatggggcttcctctcagcatcctgggggaggagctgcttctccccttaagaactagatgtgtgtgtgtctgtttggagtgatgaggaccgacccccacacccctccagcgttctgcgggtgccgaccacactgcccccggcaaaggccaggctgacttaaccttcctggtaggcctctgtagggctgggctcccagaagttttccccttaagctgcctggggatggggtggggtggagacagctccggtatctgaaatgtcactatctggggtaccgggccccctgggtgggccccactgcttccctttccctgggttcaggaaggggcttcagccccactgccctggacccccctggcctgactcccctcctgtccttccctgctccagggtcgcttggcccaaagaggtctgtggggaagctgccatggctcccacagaatcagcccacaggagacaggcatggggcccccaatctcttcactgcccttgggcgagggggtcttccttagagggaatttcgtctctaaacggtcatttctcaggcctcttgacccgacttcccaccatttctaggtgatgatgcaaacacgatgggctttccaggccgcggctcggggtccccaggaggggtcctggaggggaacgcgtggagcccttggggcttctcctggctccagtttgtcctccgcccaggaggggcacatgtgggactgtcctggccccacagcccccgtgacttcggtcctcccgggtctccacccgcccccctccatgtgtggcgggaacggccgcgctcagaggtcaggggtgtggaaagggacgagcgggggaaggttcgggaggagagaggcgcgtcccgcggcgcgcaggacgttcaccccgtgggtcccgcagcgggtctggctggggaggggcccggccgccgctc

SEQ ID NO: 9171 - RNA, 75 nt, Homo sapiens
  source 1..75: mol_type = other RNA
agaagtggctaataatattgacattattgttatagtgtcaatattattagccacttctggatttcttccatatca

SEQ ID NO: 9172 - RNA, 39 nt, Homo sapiens
  source 1..39: mol_type = other RNA
agaattgcgtttggacaatcagtggcgaagcccctgagt

SEQ ID NO: 9173 - RNA, 33 nt, Homo sapiens
  source 1..33: mol_type = other RNA
agaattgtggctggacatctgtggctgagctcc

SEQ ID NO: 9174 - RNA, 31 nt, Homo sapiens
  source 1..31: mol_type = other RNA
agacacatttggagagggaacctcccaactc

SEQ ID NO: 9175 - RNA, 35 nt, Homo sapiens
  source 1..35: mol_type = other RNA
agacacatttggagagggaccctcccaactcagat

SEQ ID NO: 9176 - RNA, 98 nt, Homo sapiens
  source 1..98: mol_type = other RNA
agacacatttggagagggaccctcccaactcagataaactgtggagagtgtaggagataggaaatggactgagaacttcctggtcccaccagagaagc

SEQ ID NO: 9177 - RNA, 4271 nt, Homo sapiens
  source 1..4271: mol_type = other RNA
agacagtagttcttgcctggtttactctgagggggaaattcaccacttatgcaggtacgagagatagcctgtcaagcactttgaagatgctggctggagacttccttctgtcttgtgatgtcatcttgcggctgatgaaattccccttgagactctctttaaagcagcttcctgctctccgcacttaatcccatgtggtataaagtaagggaggggagaagccacagatatatcaagagaaaagtaccgagaaagaaaatcagtaaagaattagagatacagagaggagaagtttttaaaaaaaaaaaaaaaaaacaggaatatgaaagagagggagctcaagtgactgaggaggcatttttaacaatcaggttatctgcaatattaaccagaaaaaaaatggtagcaaaatagagaaaatgggccatttttattccaggggacaagctgcacaaaggaatgttcttctatttattttaaacaaatgactgcgtgtactgaatctgactgtgtgaaataatctcagaatggcagcaccactggcatggcgatggtgcaggtgggtgcagttccctgtggtctctattgcttgaagagagaaagaaagttccctattattatatttaaggcagttttcagagcactggcattcttgtttgctctgttttggggatattctatttgccaatcagttcacactcatcaaccatccacttcctgtctttcacttcttcaggtgaaatatcaccactctagtgagcaccaacatggtcagagtgcaaataactgtgatggatacttcgaagtgaataagaagggaagcctgattattgctgagatcaccttggtattgccttgtacataaccaagatgtttcacagtgcctccttaagtgctcaggaaagcactttcatttaatttaatttaagctaaattctggagattttgctaaacattgacattaatgcttcatggcttttaagacaaactcatattgctaaaactatttggcagcagtaaatttatgggcagagttattgctcttacatctactgcagtacaaaactcagatgatcagcccttcgattgctcatacttattaaaataaataaataaacatgaaacatcagccacattaaggagtcagggaaactcctgaggaataacaatgtctctggagatgttttcaaatgctaacctgagactcacactgtggtttgggggtttcattattattattattattttatttcagaagaggaaagtaatattatttctcaaaataaaactttggcagagtatgaatcagggaagcagcccacacatggaaaacacaatccacaatctgaaagtagtctaggcaggctcatttttttgttgaaggaattcacatggaggcaattctgctcagttccagagagagattcttatcatcaaaagcacacacaataaccttgcttcaccacctgccactttctccagtggcctcttgttgtgaccagtaattgagaaatgacaaatgggtatagagccaaatctctaaaacagggacaccagtgtctcctagtatctgggtaataacctcctttcagtcttagtccacaccacacactaccctccagtctctcctactctttactgtcacagaaaagactctcagcttttattcacacctgccttcagaaggccaaaccattttgtgcctgaaaactgttacccactcgccccacactttacataagtatcacatatgttctttctacaaattggtatacaggtgccatttaatccattcaaatttggaagctacatcttcaagggtctgagagagctcactccccccatatattccccctttacatgttttcttataagacatacagtttaatcaattaacaaactaaacagcttatatactggcaatatattacagatgggtttatgtcagagtaatagatcacatgaaatggaccatgtggtaccccagtgcattatgtcttggtagagccctgaggacactgacagtagcatctctaagtaagtagtgctgtatgaatacagacacatgcggatctgtatctacatccatctgactaggccaaggagcaggtagatgcaagatagagacacacacatgctggatggggccactgcacaccttgtcatgccatttaaaagggcagttacaggttgccggttttgcagccattaaaattacactttatggaaaaggcttctctaattgtgtctgatttgctttctgtagtaagcatcattggaagaagaccaaagcaagagcaactagaagttaaatatacatttgagcttagctgcaatacagaaccctggggaagaagcaggctgaaagatttatttaattttaggcttggattctctcccttgctgttttcttgatgttgtgtgtctgcatttgtgtgtgtgtgtgtgtctgcgtgtgtgtgtgttccatcacatcatctcctgaagaacgctgggtttcgcaggcaggcggctagtcacctgcaacaacccaggggtcctgccgaggcttccaggctgctgtcagtgtcagatgccagggtctggtcggtggacatggaggagatgtcattgacagacgaggatggagggagactctcactgctgttcactgctgcacctgaaggagaaggctgtccttttactacaccatttttagtcttttcttctgaattcattacttccttgtagataagttctttccattcttcaattgtgtgttctctttcatccaactgcttgtcatatatctgaggtggaggcgcctccacttcggctgggtcataccagacgttgatgtagggatgctgtaaggcgtcgtccactgatattctttttgctgggtcaatcactagcatctttgacaacaagtccctggcttggctggctttgagtttattgtgctcggagtccgctgggaagagggaatctgggaagagtttggggaaggtgagtcccgcatacttgggccgattctccacatagtttcttactgtgggttgcaatttcttcatgaattctggacatggtgttcctagttgttcaattaccttattccactggtcaatatagtcccttcctggaaagaggattttgtggcgaaccatttctcccataatgcatcccacagaccatatatccacgttctccttgtagcccatccccaggatgacctcaggggctctgtaataacgtgtcaccacatatggagtcatcatgaagcttgtgcctgctgtcctggccagtccaaagtccaggattttcaatgtgcaatcagacttgactacaatgttacttggttttaaatccctgtgaataattccagcagaatggaggtgcttaatgccacacaacatttggtacagcaggtaagacattcgctcatggtctaattccatctgaatcacttgacataagttggcatccatcagttccattactaagtaaacatcttggaactcctccagcgttttctggggtgtgaagacatttaataaactaataatgtttttatggttcacacacttcatgaggaccagctcccggtacgctctcttggcatgtgtttggttctgaaagggtctgctgagcttcttaatggccacatttctgtcaaggacagcatcatacgcggcacaaactatgccctgagccccagagccaataggctttagattctggtagcgcttgagaactgtgaaggttgagtctcccacttccacactgtagaactggttgtcaactttgcttttgctcatgttgtaatgtttggcaatatatgacacatccacttgtttatcgaatccctgacaaaaggcaattttcacatccaatgttggttcactgcagtagtataagaaatggaggctcataaataccacagcttgtatggtttctcatctataggaaacgggtctaattcaacagtttcttgcataagttgccatagtgaagatctgagatgggcctgctgttggtgtttctcacactagccactgaggtggttcattagtggaacaataatgtggcaaatgctgtcctagtggtttgaacgcatttttcactctcctcctcactccctagggtcatagttttgattctgaagttagaagtgtgggggtcgtcggctgcattttcaacttggcctaaaagttggagttcaccacactgcaggcgctaggaactctgccgctcggtcaccaacctgagcctctggctagtccgaagaacgc

SEQ ID NO: 9178 - RNA, 4290 nt, Homo sapiens
  source 1..4290: mol_type = other RNA
agacagtagttcttgcctggtttactctgagggggaaattcaccacttatgcaggtacgagagatagcctgtcaagcactttgaagatgctggctggagacttccttctgtcttgtgatgtcatcttgcggctgatgaaattccccttgagactctctttaaagcagcttcctgctctccgcacttaatcccatgtggtataaagtaagggaggggagaagccacagatatatcaagagaaaagtaccgagaaagaaaatcagtaaagaattagagatacagagaggagaagtttttaaaaaaaaaaaaaaaaaacaggaatatgaaagagagggagctcaagtgactgaggaggcatttttaacaatcaggttatctgcaatattaaccagaaaaaaaatggtagcaaaatagagaaaatgggccatttttattccaggggacaagctgcacaaaggaatgttcttctatttattttaaacaaatgactgcgtgtactgaatctgactgtgtgaaataatctcagaatggcagcaccactggcatggcgatggtgcaggtgggtgcagttccctgtggtctctattgcttgaagagagaaagaaagttccctattattatatttaaggcagttttcagagcactggcattcttgtttgctctgttttggggatattctatttgccaatcagttcacactcatcaaccatccacttcctgtctttcacttcttcaggtgaaatatcaccactctagtgagcaccaacatggtcagagtgcaaataactgtgatggatacttcgaagtgaataagaagggaagcctgattattgctgagatcaccttggtattgccttgtacataaccaagatgtttcacagtgcctccttaagtgctcaggaaagcactttcatttaatttaatttaagctaaattctggagattttgctaaacattgacattaatgcttcatggcttttaagacaaactcatattgctaaaactatttggcagcagtaaatttatgggcagagttattgctcttacatctactgcagtacaaaactcagatgatcagcccttcgattgctcatacttattaaaataaataaataaacatgaaacatcagccacattaaggagtcagggaaactcctgaggaataacaatgtctctggagatgttttcaaatgctaacctgagactcacactgtggtttgggggtttcattattattattattattttatttcagaagaggaaagtaatattatttctcaaaataaaactttggcagagtatgaatcagggaagcagcccacacatggaaaacacaatccacaatctgaaagtagtctaggcaggctcatttttttgttgaaggaattcacatggaggcaattctgctcagttccagagagagattcttatcatcaaaagcacacacaataaccttgcttcaccacctgccactttctccagtggcctcttgttgtgaccagtaattgagaaatgacaaatgggtatagagccaaatctctaaaacagggacaccagtgtctcctagtatctgggtaataacctcctttcagtcttagtccacaccacacactaccctccagtctctcctactctttactgtcacagaaaagactctcagcttttattcacacctgccttcagaaggccaaaccattttgtgcctgaaaactgttacccactcgccccacactttacataagtatcacatatgttctttctacaaattggtatacaggtgccatttaatccattcaaatttggaagctacatcttcaagggtctgagagagctcactccccccatatattccccctttacatgttttcttataagacatacagtttaatcaattaacaaactaaacagcttatatactggcaatatattacagatgggtttatgtcagagtaatagatcacatgaaatggaccatgtggtaccccagtgcattatgtcttggtagagccctgaggacactgacagtagcatctctaagtaagtagtgctgtatgaatacagacacatgcggatctgtatctacatccatctgactaggccaaggagcaggtagatgcaagatagagacacacacatgctggatggggccactgcacaccttgtcatgccatttaaaagggcagttacaggttgccggttttgcagccattaaaattacactttatggaaaaggcttctctaattgtgtctgatttgctttctgtagtaagcatcattggaagaagaccaaagcaagagcaactagaagttaaatatacatttgagcttagctgcaatacagaaccctggggaagaagcaggctgaaagatttatttaattttaggcttggattctctcccttgctgttttcttgatgttgtgtgtctgcatttgtgtgtgtgtgtgtgtctgcgtgtgtgtgtgttccatcacatcatctcctgaagaacgctgggtttcgcaggcaggcggctagtcacctgcaacaacccaggggtcctgccgaggcttccaggctgctgtcagtgtcagatgccagggtctggtcggtggacatggaggagatgtcattgacagacgaggatggagggagactctcactgctgttcactgctgcacctgaaggagaaggctgtccttttactacaccatttttagtcttttcttctgaattcattacttccttgtagataagttctttccattcttcaattgtgtgttctctttcatccaactgcttgtcatatatctgaggtggaggcgcctccacttcggctgggtcataccagacgttgatgtagggatgctgtaaggcgtcgtccactgatattctttttgctgggtcaatcactagcatctttgacaacaagtccctggcttggctggctttgagtttattgtgctcggagtccgctgggaagagggaatctgggaagagtttggggaaggtgagtcccgcatacttgggccgattctccacatagtttcttactgtgggttgcaatttcttcatgaattctggacatggtgttcctagttgttcaattaccttattccactggtcaatatagtcccttcctggaaagaggattttgtggcgaaccatttctcccataatgcatcccacagaccatatatccacgttctccttgtagcccatccccaggatgacctcaggggctctgtaataacgtgtcaccacatatggagtcatcatgaagcttgtgcctgctgtcctggccagtccaaagtccaggattttcaatgtgcaatcagacttgactacaatgttacttggttttaaatccctgtgaataattccagcagaatggaggtgcttaatgccacacaacatttggtacagcaggtaagacattcgctcatggtctaattccatctgaatcacttgacataagttggcatccatcagttccattactaagtaaacatcttggaactcctccagcgttttctggggtgtgaagacatttaataaactaataatgtttttatggttcacacacttcatgaggaccagctcccggtacgctctcttggcatgtgtttggttctgaaagggtctgctgagcttcttaatggccacatttctgtcaaggacagcatcatacgcggcacaaactatgccctgagccccagagccaataggctttagattctggtagcgcttgagaactgtgaaggttgagtctcccacttccacactgtagaactggttgtcaactttgcttttgctcatgttgtaatgtttggcaatatatgacacatccacttgtttatcgaatccctgacaaaaggcaattttcacatccaatgttggttcactgcagtagtataagaaatggaggctcataaataccacagcttgtatggtttctcatctataggaaacgggtctaattcaacagtttcttgcataagttgccatagtgaagatctgagatgggcctgctgttggtgtttctcacactagccagacaatgacagcaaaaacacactcagcccctctgggatctgttcataaacatccccttccagcatggcaaacacactcctctcaacagcagatgctgttctggggctagcaggcaggaagctggaggcagctgattttcccactctacatataatttcttactgcctcactatccagaatcgttttactgaaactgtgaggattttttaagaacaggagcccctcaaattaaagacactttgcaacagcagaggaa

SEQ ID NO: 9179 - RNA, 4821 nt, Homo sapiens
  source 1..4821: mol_type = other RNA
agacagtagttcttgcctggtttactctgagggggaaattcaccacttatgcaggtacgagagatagcctgtcaagcactttgaagatgctggctggagacttccttctgtcttgtgatgtcatcttgcggctgatgaaattccccttgagactctctttaaagcagcttcctgctctccgcacttaatcccatgtggtataaagtaagggaggggagaagccacagatatatcaagagaaaagtaccgagaaagaaaatcagtaaagaattagagatacagagaggagaagtttttaaaaaaaaaaaaaaaaaacaggaatatgaaagagagggagctcaagtgactgaggaggcatttttaacaatcaggttatctgcaatattaaccagaaaaaaaatggtagcaaaatagagaaaatgggccatttttattccaggggacaagctgcacaaaggaatgttcttctatttattttaaacaaatgactgcgtgtactgaatctgactgtgtgaaataatctcagaatggcagcaccactggcatggcgatggtgcaggtgggtgcagttccctgtggtctctattgcttgaagagagaaagaaagttccctattattatatttaaggcagttttcagagcactggcattcttgtttgctctgttttggggatattctatttgccaatcagttcacactcatcaaccatccacttcctgtctttcacttcttcaggtgaaatatcaccactctagtgagcaccaacatggtcagagtgcaaataactgtgatggatacttcgaagtgaataagaagggaagcctgattattgctgagatcaccttggtattgccttgtacataaccaagatgtttcacagtgcctccttaagtgctcaggaaagcactttcatttaatttaatttaagctaaattctggagattttgctaaacattgacattaatgcttcatggcttttaagacaaactcatattgctaaaactatttggcagcagtaaatttatgggcagagttattgctcttacatctactgcagtacaaaactcagatgatcagcccttcgattgctcatacttattaaaataaataaataaacatgaaacatcagccacattaaggagtcagggaaactcctgaggaataacaatgtctctggagatgttttcaaatgctaacctgagactcacactgtggtttgggggtttcattattattattattattttatttcagaagaggaaagtaatattatttctcaaaataaaactttggcagagtatgaatcagggaagcagcccacacatggaaaacacaatccacaatctgaaagtagtctaggcaggctcatttttttgttgaaggaattcacatggaggcaattctgctcagttccagagagagattcttatcatcaaaagcacacacaataaccttgcttcaccacctgccactttctccagtggcctcttgttgtgaccagtaattgagaaatgacaaatgggtatagagccaaatctctaaaacagggacaccagtgtctcctagtatctgggtaataacctcctttcagtcttagtccacaccacacactaccctccagtctctcctactctttactgtcacagaaaagactctcagcttttattcacacctgccttcagaaggccaaaccattttgtgcctgaaaactgttacccactcgccccacactttacataagtatcacatatgttctttctacaaattggtatacaggtgccatttaatccattcaaatttggaagctacatcttcaagggtctgagagagctcactccccccatatattccccctttacatgttttcttataagacatacagtttaatcaattaacaaactaaacagcttatatactggcaatatattacagatgggtttatgtcagagtaatagatcacatgaaatggaccatgtggtaccccagtgcattatgtcttggtagagccctgaggacactgacagtagcatctctaagtaagtagtgctgtatgaatacagacacatgcggatctgtatctacatccatctgactaggccaaggagcaggtagatgcaagatagagacacacacatgctggatggggccactgcacaccttgtcatgccatttaaaagggcagttacaggttgccggttttgcagccattaaaattacactttatggaaaaggcttctctaattgtgtctgatttgctttctgtagtaagcatcattggaagaagaccaaagcaagagcaactagaagttaaatatacatttgagcttagctgcaatacagaaccctggggaagaagcaggctgaaagatttatttaattttaggcttggattctctcccttgctgttttcttgatgttgtgtgtctgcatttgtgtgtgtgtgtgtgtctgcgtgtgtgtgtgttccatcacatcatctcctgaagaacgctgggtttcgcaggcaggcggctagtcacctgcaacaacccaggggtcctgccgaggcttccaggctgctgtcagtgtcagatgccagggtctggtcggtggacatggaggagatgtcattgacagacgaggatggagggagactctcactgctgttcactgctgcacctgaaggagaaggctgtccttttactacaccatttttagtcttttcttctgaattcattacttccttgtagataagttctttccattcttcaattgtgtgttctctttcatccaactgcttgtcatatatctgaggtggaggcgcctccacttcggctgggtcataccagacgttgatgtagggatgctgtaaggcgtcgtccactgatattctttttgctgggtcaatcactagcatctttgacaacaagtccctggcttggctggctttgagtttattgtgctcggagtccgctgggaagagggaatctgggaagagtttggggaaggtgagtcccgcatacttgggccgattctccacatagtttcttactgtgggttgcaatttcttcatgaattctggacatggtgttcctagttgttcaattaccttattccactggtcaatatagtcccttcctggaaagaggattttgtggcgaaccatttctcccataatgcatcccacagaccatatatccacgttctccttgtagcccatccccaggatgacctcaggggctctgtaataacgtgtcaccacatatggagtcatcatgaagcttgtgcctgctgtcctggccagtccaaagtccaggattttcaatgtgcaatcagacttgactacaatgttacttggttttaaatccctgtgaataattccagcagaatggaggtgcttaatgccacacaacatttggtacagcaggtaagacattcgctcatggtctaattccatctgaatcacttgacataagttggcatccatcagttccattactaagtaaacatcttggaactcctccagcgttttctggggtgtgaagacatttaataaactaataatgtttttatggttcacacacttcatgaggaccagctcccggtacgctctcttggcatgtgtttggttctgaaagggtctgctgagcttcttaatggccacatttctgtcaaggacagcatcatacgcggcacaaactatgccctgagccccagagccaataggctttagattctggtagcgcttgagaactgtgaaggttgagtctcccacttccacactgtagaactggttgtcaactttgcttttgctcatgttgtaatgtttggcaatatatgacacatccacttgtttatcgaatccctgacaaaaggcaattttcacatccaatgttggttcactgcagtagtataagaaatggaggctcataaataccacagcttgtatggtttctcatctataggaaacgggtctaattcaacagtttcttgcataagttgccatagtgaagatctgagatgggcctgctgttggtgtttctcacactagccagaggcagccaaaccgctacatccaaagcatccagcccctaaaatctaatggttctgaagtggagtcagaagcttgtgatatacttatatatttatttgttatatatttgtaacatatatgctcacctaaagtagaaaattcacagaagcttctctgagagaaatggtccttactgcaactattttaaatatgttgataagcattctgtgttatcttccagggtccgacaactagccgatgagggatagaaggagatattggatgttgtgctggcaatgcctggtgcacttacactcgttttccttccacctgaactgtagtctatcccatatgacttagcctgcttccttgcagtttgttcataaaagttatcatcaacatggccagaagcaggcagggctgctgtacagacactgtcaggctctgcaccaaaggcagcccatgtaaacaaccttgtgattgcttcagagcctactgctgtggcataagccattctttttctgtggctaaattgcagtaccctgggaagttatctgtttaagggggtaaaagcagagactaggtctctagatttaaatgtttggggagggtgagaaaaatatatggatagatagttttcttgtaatatctatagcctgatttacttacagattttccagtaaattacatttattttgttgaaggcacaaatacatagattctaacaaatatactgccatacttatttctgatttttttttcaaaagagctctgacatttgcaggggacacagtatcccagcacagaa

SEQ ID NO: 9180 - RNA, 4428 nt, Homo sapiens
  source 1..4428: mol_type = other RNA
agacagtagttcttgcctggtttactctgagggggaaattcaccacttatgcaggtacgagagatagcctgtcaagcactttgaagatgctggctggagacttccttctgtcttgtgatgtcatcttgcggctgatgaaattccccttgagactctctttaaagcagcttcctgctctccgcacttaatcccatgtggtataaagtaagggaggggagaagccacagatatatcaagagaaaagtaccgagaaagaaaatcagtaaagaattagagatacagagaggagaagtttttaaaaaaaaaaaaaaaaaacaggaatatgaaagagagggagctcaagtgactgaggaggcatttttaacaatcaggttatctgcaatattaaccagaaaaaaaatggtagcaaaatagagaaaatgggccatttttattccaggggacaagctgcacaaaggaatgttcttctatttattttaaacaaatgactgcgtgtactgaatctgactgtgtgaaataatctcagaatggcagcaccactggcatggcgatggtgcaggtgggtgcagttccctgtggtctctattgcttgaagagagaaagaaagttccctattattatatttaaggcagttttcagagcactggcattcttgtttgctctgttttggggatattctatttgccaatcagttcacactcatcaaccatccacttcctgtctttcacttcttcaggtgaaatatcaccactctagtgagcaccaacatggtcagagtgcaaataactgtgatggatacttcgaagtgaataagaagggaagcctgattattgctgagatcaccttggtattgccttgtacataaccaagatgtttcacagtgcctccttaagtgctcaggaaagcactttcatttaatttaatttaagctaaattctggagattttgctaaacattgacattaatgcttcatggcttttaagacaaactcatattgctaaaactatttggcagcagtaaatttatgggcagagttattgctcttacatctactgcagtacaaaactcagatgatcagcccttcgattgctcatacttattaaaataaataaataaacatgaaacatcagccacattaaggagtcagggaaactcctgaggaataacaatgtctctggagatgttttcaaatgctaacctgagactcacactgtggtttgggggtttcattattattattattattttatttcagaagaggaaagtaatattatttctcaaaataaaactttggcagagtatgaatcagggaagcagcccacacatggaaaacacaatccacaatctgaaagtagtctaggcaggctcatttttttgttgaaggaattcacatggaggcaattctgctcagttccagagagagattcttatcatcaaaagcacacacaataaccttgcttcaccacctgccactttctccagtggcctcttgttgtgaccagtaattgagaaatgacaaatgggtatagagccaaatctctaaaacagggacaccagtgtctcctagtatctgggtaataacctcctttcagtcttagtccacaccacacactaccctccagtctctcctactctttactgtcacagaaaagactctcagcttttattcacacctgccttcagaaggccaaaccattttgtgcctgaaaactgttacccactcgccccacactttacataagtatcacatatgttctttctacaaattggtatacaggtgccatttaatccattcaaatttggaagctacatcttcaagggtctgagagagctcactccccccatatattccccctttacatgttttcttataagacatacagtttaatcaattaacaaactaaacagcttatatactggcaatatattacagatgggtttatgtcagagtaatagatcacatgaaatggaccatgtggtaccccagtgcattatgtcttggtagagccctgaggacactgacagtagcatctctaagtaagtagtgctgtatgaatacagacacatgcggatctgtatctacatccatctgactaggccaaggagcaggtagatgcaagatagagacacacacatgctggatggggccactgcacaccttgtcatgccatttaaaagggcagttacaggttgccggttttgcagccattaaaattacactttatggaaaaggcttctctaattgtgtctgatttgctttctgtagtaagcatcattggaagaagaccaaagcaagagcaactagaagttaaatatacatttgagcttagctgcaatacagaaccctggggaagaagcaggctgaaagatttatttaattttaggcttggattctctcccttgctgttttcttgatgttgtgtgtctgcatttgtgtgtgtgtgtgtgtctgcgtgtgtgtgtgttccatcacatcatctcctgaagaacgctgggtttcgcaggcaggcggctagtcacctgcaacaacccaggggtcctgccgaggcttccaggctgctgtcagtgtcagatgccagggtctggtcggtggacatggaggagatgtcattgacagacgaggatggagggagactctcactgctgttcactgctgcacctgaaggagaaggctgtccttttactacaccatttttagtcttttcttctgaattcattacttccttgtagataagttctttccattcttcaattgtgtgttctctttcatccaactgcttgtcatatatctgaggtggaggcgcctccacttcggctgggtcataccagacgttgatgtagggatgctgtaaggcgtcgtccactgatattctttttgctgggtcaatcactagcatctttgacaacaagtccctggcttggctggctttgagtttattgtgctcggagtccgctgggaagagggaatctgggaagagtttggggaaggtgagtcccgcatacttgggccgattctccacatagtttcttactgtgggttgcaatttcttcatgaattctggacatggtgttcctagttgttcaattaccttattccactggtcaatatagtcccttcctggaaagaggattttgtggcgaaccatttctcccataatgcatcccacagaccatatatccacgttctccttgtagcccatccccaggatgacctcaggggctctgtaataacgtgtcaccacatatggagtcatcatgaagcttgtgcctgctgtcctggccagtccaaagtccaggattttcaatgtgcaatcagacttgactacaatgttacttggttttaaatccctgtgaataattccagcagaatggaggtgcttaatgccacacaacatttggtacagcaggtaagacattcgctcatggtctaattccatctgaatcacttgacataagttggcatccatcagttccattactaagtaaacatcttggaactcctccagcgttttctggggtgtgaagacatttaataaactaataatgtttttatggttcacacacttcatgaggaccagctcccggtacgctctcttggcatgtgtttggttctgaaagggtctgctgagcttcttaatggccacatttctgtcaaggacagcatcatacgcggcacaaactatgccctgagccccagagccaataggctttagattctggtagcgcttgagaactgtgaaggttgagtctcccacttccacactgtagaactggttgtcaactttgcttttgctcatgttgtaatgtttggcaatatatgacacatccacttgtttatcgaatccctgacaaaaggcaattttcacatccaatgttggttcactgcagtagtataagaaatggaggctcataaataccacagcttgtatggtttctcatctataggaaacgggtctaattcaacagtttcttgcataagttgccatagtgaagatctgagatgggcctgctgttggtgtttctcacactagccattccgtgcctgagaactacgatcctgatccggcagtgtttgccccagaaatcctccctacttgtttttcattaaccacattccagactaacatggaagagattctttggagatatggagattgtttaaaattaacgatggacaggtgatttccaagaaaacccaatcttaaactcactcaagcccctaggaattgaggggtgaggacaaaaaaggaaatttgtaaaaatgaaaaaagaaaagaaaaaggtaagcatatagcaagcaccacccacccccataaaaataaaaagtgaaggggaggttaaagaaaatagaagaagagtggcttgctgaatcaccctctttcactgcctggaaaccattgtgcagcgtgatgctgcctgtaccattgt

SEQ ID NO: 9181 - RNA, 4199 nt, Homo sapiens
  source 1..4199: mol_type = other RNA
agacagtagttcttgcctggtttactctgagggggaaattcaccacttatgcaggtacgagagatagcctgtcaagcactttgaagatgctggctggagacttccttctgtcttgtgatgtcatcttgcggctgatgaaattccccttgagactctctttaaagcagcttcctgctctccgcacttaatcccatgtggtataaagtaagggaggggagaagccacagatatatcaagagaaaagtaccgagaaagaaaatcagtaaagaattagagatacagagaggagaagtttttaaaaaaaaaaaaaaaaaacaggaatatgaaagagagggagctcaagtgactgaggaggcatttttaacaatcaggttatctgcaatattaaccagaaaaaaaatggtagcaaaatagagaaaatgggccatttttattccaggggacaagctgcacaaaggaatgttcttctatttattttaaacaaatgactgcgtgtactgaatctgactgtgtgaaataatctcagaatggcagcaccactggcatggcgatggtgcaggtgggtgcagttccctgtggtctctattgcttgaagagagaaagaaagttccctattattatatttaaggcagttttcagagcactggcattcttgtttgctctgttttggggatattctatttgccaatcagttcacactcatcaaccatccacttcctgtctttcacttcttcaggtgaaatatcaccactctagtgagcaccaacatggtcagagtgcaaataactgtgatggatacttcgaagtgaataagaagggaagcctgattattgctgagatcaccttggtattgccttgtacataaccaagatgtttcacagtgcctccttaagtgctcaggaaagcactttcatttaatttaatttaagctaaattctggagattttgctaaacattgacattaatgcttcatggcttttaagacaaactcatattgctaaaactatttggcagcagtaaatttatgggcagagttattgctcttacatctactgcagtacaaaactcagatgatcagcccttcgattgctcatacttattaaaataaataaataaacatgaaacatcagccacattaaggagtcagggaaactcctgaggaataacaatgtctctggagatgttttcaaatgctaacctgagactcacactgtggtttgggggtttcattattattattattattttatttcagaagaggaaagtaatattatttctcaaaataaaactttggcagagtatgaatcagggaagcagcccacacatggaaaacacaatccacaatctgaaagtagtctaggcaggctcatttttttgttgaaggaattcacatggaggcaattctgctcagttccagagagagattcttatcatcaaaagcacacacaataaccttgcttcaccacctgccactttctccagtggcctcttgttgtgaccagtaattgagaaatgacaaatgggtatagagccaaatctctaaaacagggacaccagtgtctcctagtatctgggtaataacctcctttcagtcttagtccacaccacacactaccctccagtctctcctactctttactgtcacagaaaagactctcagcttttattcacacctgccttcagaaggccaaaccattttgtgcctgaaaactgttacccactcgccccacactttacataagtatcacatatgttctttctacaaattggtatacaggtgccatttaatccattcaaatttggaagctacatcttcaagggtctgagagagctcactccccccatatattccccctttacatgttttcttataagacatacagtttaatcaattaacaaactaaacagcttatatactggcaatatattacagatgggtttatgtcagagtaatagatcacatgaaatggaccatgtggtaccccagtgcattatgtcttggtagagccctgaggacactgacagtagcatctctaagtaagtagtgctgtatgaatacagacacatgcggatctgtatctacatccatctgactaggccaaggagcaggtagatgcaagatagagacacacacatgctggatggggccactgcacaccttgtcatgccatttaaaagggcagttacaggttgccggttttgcagccattaaaattacactttatggaaaaggcttctctaattgtgtctgatttgctttctgtagtaagcatcattggaagaagaccaaagcaagagcaactagaagttaaatatacatttgagcttagctgcaatacagaaccctggggaagaagcaggctgaaagatttatttaattttaggcttggattctctcccttgctgttttcttgatgttgtgtgtctgcatttgtgtgtgtgtgtgtgtctgcgtgtgtgtgtgttccatcacatcatctcctgaagaacgctgggtttcgcaggcaggcggctagtcacctgcaacaacccaggggtcctgccgaggcttccaggctgctgtcagtgtcagatgccagggtctggtcggtggacatggaggagatgtcattgacagacgaggatggagggagactctcactgctgttcactgctgcacctgaaggagaaggctgtccttttactacaccatttttagtcttttcttctgaattcattacttccttgtagataagttctttccattcttcaattgtgtgttctctttcatccaactgcttgtcatatatctgaggtggaggcgcctccacttcggctgggtcataccagacgttgatgtagggatgctgtaaggcgtcgtccactgatattctttttgctgggtcaatcactagcatctttgacaacaagtccctggcttggctggctttgagtttattgtgctcggagtccgctgggaagagggaatctgggaagagtttggggaaggtgagtcccgcatacttgggccgattctccacatagtttcttactgtgggttgcaatttcttcatgaattctggacatggtgttcctagttgttcaattaccttattccactggtcaatatagtcccttcctggaaagaggattttgtggcgaaccatttctcccataatgcatcccacagaccatatatccacgttctccttgtagcccatccccaggatgacctcaggggctctgtaataacgtgtcaccacatatggagtcatcatgaagcttgtgcctgctgtcctggccagtccaaagtccaggattttcaatgtgcaatcagacttgactacaatgttacttggttttaaatccctgtgaataattccagcagaatggaggtgcttaatgccacacaacatttggtacagcaggtaagacattcgctcatggtctaattccatctgaatcacttgacataagttggcatccatcagttccattactaagtaaacatcttggaactcctccagcgttttctggggtgtgaagacatttaataaactaataatgtttttatggttcacacacttcatgaggaccagctcccggtacgctctcttggcatgtgtttggttctgaaagggtctgctgagcttcttaatggccacatttctgtcaaggacagcatcatacgcggcacaaactatgccctgagccccagagccaataggctttagattctggtagcgcttgagaactgtgaaggttgagtctcccacttccacactgtagaactggttgtcaactttgcttttgctcatgttgtaatgtttggcaatatatgacacatccacttgtttatcgaatccctgacaaaaggcaattttcacatccaatgttggttcactgcagtagtataagaaatggaggctcataaataccacagcttgtatggtttctcatctataggaaacgggtctaattcaacagtttcttgcataagttgccatagtgaagatctgagatgggcctgctgttggtgtttctcacactagcctaaagtagaaaattcacagaagcttctctgagagaaatggtccttactgcaactattttaaatatgttgataagcattctgtgttatcttccagggtccgacaactagccgatgagggatagaaggagatattggatgttgtgctggcaatgcctggtgcacttac

SEQ ID NO: 9182 - RNA, 4194 nt, Homo sapiens
  source 1..4194: mol_type = other RNA
agacagtagttcttgcctggtttactctgagggggaaattcaccacttatgcaggtacgagagatagcctgtcaagcactttgaagatgctggctggagacttccttctgtcttgtgatgtcatcttgcggctgatgaaattccccttgagactctctttaaagcagcttcctgctctccgcacttaatcccatgtggtataaagtaagggaggggagaagccacagatatatcaagagaaaagtaccgagaaagaaaatcagtaaagaattagagatacagagaggagaagtttttaaaaaaaaaaaaaaaaaacaggaatatgaaagagagggagctcaagtgactgaggaggcatttttaacaatcaggttatctgcaatattaaccagaaaaaaaatggtagcaaaatagagaaaatgggccatttttattccaggggacaagctgcacaaaggaatgttcttctatttattttaaacaaatgactgcgtgtactgaatctgactgtgtgaaataatctcagaatggcagcaccactggcatggcgatggtgcaggtgggtgcagttccctgtggtctctattgcttgaagagagaaagaaagttccctattattatatttaaggcagttttcagagcactggcattcttgtttgctctgttttggggatattctatttgccaatcagttcacactcatcaaccatccacttcctgtctttcacttcttcaggtgaaatatcaccactctagtgagcaccaacatggtcagagtgcaaataactgtgatggatacttcgaagtgaataagaagggaagcctgattattgctgagatcaccttggtattgccttgtacataaccaagatgtttcacagtgcctccttaagtgctcaggaaagcactttcatttaatttaatttaagctaaattctggagattttgctaaacattgacattaatgcttcatggcttttaagacaaactcatattgctaaaactatttggcagcagtaaatttatgggcagagttattgctcttacatctactgcagtacaaaactcagatgatcagcccttcgattgctcatacttattaaaataaataaataaacatgaaacatcagccacattaaggagtcagggaaactcctgaggaataacaatgtctctggagatgttttcaaatgctaacctgagactcacactgtggtttgggggtttcattattattattattattttatttcagaagaggaaagtaatattatttctcaaaataaaactttggcagagtatgaatcagggaagcagcccacacatggaaaacacaatccacaatctgaaagtagtctaggcaggctcatttttttgttgaaggaattcacatggaggcaattctgctcagttccagagagagattcttatcatcaaaagcacacacaataaccttgcttcaccacctgccactttctccagtggcctcttgttgtgaccagtaattgagaaatgacaaatgggtatagagccaaatctctaaaacagggacaccagtgtctcctagtatctgggtaataacctcctttcagtcttagtccacaccacacactaccctccagtctctcctactctttactgtcacagaaaagactctcagcttttattcacacctgccttcagaaggccaaaccattttgtgcctgaaaactgttacccactcgccccacactttacataagtatcacatatgttctttctacaaattggtatacaggtgccatttaatccattcaaatttggaagctacatcttcaagggtctgagagagctcactccccccatatattccccctttacatgttttcttataagacatacagtttaatcaattaacaaactaaacagcttatatactggcaatatattacagatgggtttatgtcagagtaatagatcacatgaaatggaccatgtggtaccccagtgcattatgtcttggtagagccctgaggacactgacagtagcatctctaagtaagtagtgctgtatgaatacagacacatgcggatctgtatctacatccatctgactaggccaaggagcaggtagatgcaagatagagacacacacatgctggatggggccactgcacaccttgtcatgccatttaaaagggcagttacaggttgccggttttgcagccattaaaattacactttatggaaaaggcttctctaattgtgtctgatttgctttctgtagtaagcatcattggaagaagaccaaagcaagagcaactagaagttaaatatacatttgagcttagctgcaatacagaaccctggggaagaagcaggctgaaagatttatttaattttaggcttggattctctcccttgctgttttcttgatgttgtgtgtctgcatttgtgtgtgtgtgtgtgtctgcgtgtgtgtgtgttccatcacatcatctcctgaagaacgctgggtttcgcaggcaggcggctagtcacctgcaacaacccaggggtcctgccgaggcttccaggctgctgtcagtgtcagatgccagggtctggtcggtggacatggaggagatgtcattgacagacgaggatggagggagactctcactgctgttcactgctgcacctgaaggagaaggctgtccttttactacaccatttttagtcttttcttctgaattcattacttccttgtagataagttctttccattcttcaattgtgtgttctctttcatccaactgcttgtcatatatctgaggtggaggcgcctccacttcggctgggtcataccagacgttgatgtagggatgctgtaaggcgtcgtccactgatattctttttgctgggtcaatcactagcatctttgacaacaagtccctggcttggctggctttgagtttattgtgctcggagtccgctgggaagagggaatctgggaagagtttggggaaggtgagtcccgcatacttgggccgattctccacatagtttcttactgtgggttgcaatttcttcatgaattctggacatggtgttcctagttgttcaattaccttattccactggtcaatatagtcccttcctggaaagaggattttgtggcgaaccatttctcccataatgcatcccacagaccatatatccacgttctccttgtagcccatccccaggatgacctcaggggctctgtaataacgtgtcaccacatatggagtcatcatgaagcttgtgcctgctgtcctggccagtccaaagtccaggattttcaatgtgcaatcagacttgactacaatgttacttggttttaaatccctgtgaataattccagcagaatggaggtgcttaatgccacacaacatttggtacagcaggtaagacattcgctcatggtctaattccatctgaatcacttgacataagttggcatccatcagttccattactaagtaaacatcttggaactcctccagcgttttctggggtgtgaagacatttaataaactaataatgtttttatggttcacacacttcatgaggaccagctcccggtacgctctcttggcatgtgtttggttctgaaagggtctgctgagcttcttaatggccacatttctgtcaaggacagcatcatacgcggcacaaactatgccctgagccccagagccaataggctttagattctggtagcgcttgagaactgtgaaggttgagtctcccacttccacactgtagaactggttgtcaactttgcttttgctcatgttgtaatgtttggcaatatatgacacatccacttgtttatcgaatccctgacaaaaggcaattttcacatccaatgttggttcactgcagtagtataagaaatggaggctcataaataccacagcttgtatggtttctcatctataggaaacgggtctaattcaacagtttcttgcataagttgccatagtgaagatctgagatgggcctgctgttggtgtttctcacactagcctgatgtctcctcttaagagtttctaccaagattcacaataagaaatacagcttctccctattaaatacagaaaacaaaagatatgcaaaacacaggttttgtattttccccttctttgccttgatcggttcatgaggataaaatgtactcaaactgaaaaa

SEQ ID NO: 9183 - RNA, 4382 nt, Homo sapiens
  source 1..4382: mol_type = other RNA
agacagtagttcttgcctggtttactctgagggggaaattcaccacttatgcaggtacgagagatagcctgtcaagcactttgaagatgctggctggagacttccttctgtcttgtgatgtcatcttgcggctgatgaaattccccttgagactctctttaaagcagcttcctgctctccgcacttaatcccatgtggtataaagtaagggaggggagaagccacagatatatcaagagaaaagtaccgagaaagaaaatcagtaaagaattagagatacagagaggagaagtttttaaaaaaaaaaaaaaaaaacaggaatatgaaagagagggagctcaagtgactgaggaggcatttttaacaatcaggttatctgcaatattaaccagaaaaaaaatggtagcaaaatagagaaaatgggccatttttattccaggggacaagctgcacaaaggaatgttcttctatttattttaaacaaatgactgcgtgtactgaatctgactgtgtgaaataatctcagaatggcagcaccactggcatggcgatggtgcaggtgggtgcagttccctgtggtctctattgcttgaagagagaaagaaagttccctattattatatttaaggcagttttcagagcactggcattcttgtttgctctgttttggggatattctatttgccaatcagttcacactcatcaaccatccacttcctgtctttcacttcttcaggtgaaatatcaccactctagtgagcaccaacatggtcagagtgcaaataactgtgatggatacttcgaagtgaataagaagggaagcctgattattgctgagatcaccttggtattgccttgtacataaccaagatgtttcacagtgcctccttaagtgctcaggaaagcactttcatttaatttaatttaagctaaattctggagattttgctaaacattgacattaatgcttcatggcttttaagacaaactcatattgctaaaactatttggcagcagtaaatttatgggcagagttattgctcttacatctactgcagtacaaaactcagatgatcagcccttcgattgctcatacttattaaaataaataaataaacatgaaacatcagccacattaaggagtcagggaaactcctgaggaataacaatgtctctggagatgttttcaaatgctaacctgagactcacactgtggtttgggggtttcattattattattattattttatttcagaagaggaaagtaatattatttctcaaaataaaactttggcagagtatgaatcagggaagcagcccacacatggaaaacacaatccacaatctgaaagtagtctaggcaggctcatttttttgttgaaggaattcacatggaggcaattctgctcagttccagagagagattcttatcatcaaaagcacacacaataaccttgcttcaccacctgccactttctccagtggcctcttgttgtgaccagtaattgagaaatgacaaatgggtatagagccaaatctctaaaacagggacaccagtgtctcctagtatctgggtaataacctcctttcagtcttagtccacaccacacactaccctccagtctctcctactctttactgtcacagaaaagactctcagcttttattcacacctgccttcagaaggccaaaccattttgtgcctgaaaactgttacccactcgccccacactttacataagtatcacatatgttctttctacaaattggtatacaggtgccatttaatccattcaaatttggaagctacatcttcaagggtctgagagagctcactccccccatatattccccctttacatgttttcttataagacatacagtttaatcaattaacaaactaaacagcttatatactggcaatatattacagatgggtttatgtcagagtaatagatcacatgaaatggaccatgtggtaccccagtgcattatgtcttggtagagccctgaggacactgacagtagcatctctaagtaagtagtgctgtatgaatacagacacatgcggatctgtatctacatccatctgactaggccaaggagcaggtagatgcaagatagagacacacacatgctggatggggccactgcacaccttgtcatgccatttaaaagggcagttacaggttgccggttttgcagccattaaaattacactttatggaaaaggcttctctaattgtgtctgatttgctttctgtagtaagcatcattggaagaagaccaaagcaagagcaactagaagttaaatatacatttgagcttagctgcaatacagaaccctggggaagaagcaggctgaaagatttatttaattttaggcttggattctctcccttgctgttttcttgatgttgtgtgtctgcatttgtgtgtgtgtgtgtgtctgcgtgtgtgtgtgttccatcacatcatctcctgaagaacgctgggtttcgcaggcaggcggctagtcacctgcaacaacccaggggtcctgccgaggcttccaggctgctgtcagtgtcagatgccagggtctggtcggtggacatggaggagatgtcattgacagacgaggatggagggagactctcactgctgttcactgctgcacctgaaggagaaggctgtccttttactacaccatttttagtcttttcttctgaattcattacttccttgtagataagttctttccattcttcaattgtgtgttctctttcatccaactgcttgtcatatatctgaggtggaggcgcctccacttcggctgggtcataccagacgttgatgtagggatgctgtaaggcgtcgtccactgatattctttttgctgggtcaatcactagcatctttgacaacaagtccctggcttggctggctttgagtttattgtgctcggagtccgctgggaagagggaatctgggaagagtttggggaaggtgagtcccgcatacttgggccgattctccacatagtttcttactgtgggttgcaatttcttcatgaattctggacatggtgttcctagttgttcaattaccttattccactggtcaatatagtcccttcctggaaagaggattttgtggcgaaccatttctcccataatgcatcccacagaccatatatccacgttctccttgtagcccatccccaggatgacctcaggggctctgtaataacgtgtcaccacatatggagtcatcatgaagcttgtgcctgctgtcctggccagtccaaagtccaggattttcaatgtgcaatcagacttgactacaatgttacttggttttaaatccctgtgaataattccagcagaatggaggtgcttaatgccacacaacatttggtacagcaggtaagacattcgctcatggtctaattccatctgaatcacttgacataagttggcatccatcagttccattactaagtaaacatcttggaactcctccagcgttttctggggtgtgaagacatttaataaactaataatgtttttatggttcacacacttcatgaggaccagctcccggtacgctctcttggcatgtgtttggttctgaaagggtctgctgagcttcttaatggccacatttctgtcaaggacagcatcatacgcggcacaaactatgccctgagccccagagccaataggctttagattctggtagcgcttgagaactgtgaaggttgagtctcccacttccacactgtagaactggttgtcaactttgcttttgctcatgttgtaatgtttggcaatatatgacacatccacttgtttatcgaatccctgacaaaaggcaattttcacatccaatgttggttcactgcagtagtataagaaatggaggctcataaataccacagcttgtatggtttctcatctataggaaacgggtctaattcaacagtttcttgcataagttgccatagtgaagatctgagatgggcctgctgttggtgtttctcacactagcctggagctgagtcaatttagagagctgcgtgaaatacaggggtagaggaagcagcggcaaaatccctctgggctcgctgggtcccctgccacgccatttctgcctggcctcacaggggtccttgaggagggctgctggaggcactgggaaagctgcagggagaaggaaaactccagctgaactttgtaacaatttcaactgatggagaagtctcttggccagaactcagggggagggcatgaatccagtgtgcagactcaacagagcagggaagaaggagagccctgtttattttcacagctgggaggcgggtagcctggggaaagtactcggtcctgcttgcccactgc

SEQ ID NO: 9184 - RNA, 4900 nt, Homo sapiens
  source 1..4900: mol_type = other RNA
agacagtagttcttgcctggtttactctgagggggaaattcaccacttatgcaggtacgagagatagcctgtcaagcactttgaagatgctggctggagacttccttctgtcttgtgatgtcatcttgcggctgatgaaattccccttgagactctctttaaagcagcttcctgctctccgcacttaatcccatgtggtataaagtaagggaggggagaagccacagatatatcaagagaaaagtaccgagaaagaaaatcagtaaagaattagagatacagagaggagaagtttttaaaaaaaaaaaaaaaaaacaggaatatgaaagagagggagctcaagtgactgaggaggcatttttaacaatcaggttatctgcaatattaaccagaaaaaaaatggtagcaaaatagagaaaatgggccatttttattccaggggacaagctgcacaaaggaatgttcttctatttattttaaacaaatgactgcgtgtactgaatctgactgtgtgaaataatctcagaatggcagcaccactggcatggcgatggtgcaggtgggtgcagttccctgtggtctctattgcttgaagagagaaagaaagttccctattattatatttaaggcagttttcagagcactggcattcttgtttgctctgttttggggatattctatttgccaatcagttcacactcatcaaccatccacttcctgtctttcacttcttcaggtgaaatatcaccactctagtgagcaccaacatggtcagagtgcaaataactgtgatggatacttcgaagtgaataagaagggaagcctgattattgctgagatcaccttggtattgccttgtacataaccaagatgtttcacagtgcctccttaagtgctcaggaaagcactttcatttaatttaatttaagctaaattctggagattttgctaaacattgacattaatgcttcatggcttttaagacaaactcatattgctaaaactatttggcagcagtaaatttatgggcagagttattgctcttacatctactgcagtacaaaactcagatgatcagcccttcgattgctcatacttattaaaataaataaataaacatgaaacatcagccacattaaggagtcagggaaactcctgaggaataacaatgtctctggagatgttttcaaatgctaacctgagactcacactgtggtttgggggtttcattattattattattattttatttcagaagaggaaagtaatattatttctcaaaataaaactttggcagagtatgaatcagggaagcagcccacacatggaaaacacaatccacaatctgaaagtagtctaggcaggctcatttttttgttgaaggaattcacatggaggcaattctgctcagttccagagagagattcttatcatcaaaagcacacacaataaccttgcttcaccacctgccactttctccagtggcctcttgttgtgaccagtaattgagaaatgacaaatgggtatagagccaaatctctaaaacagggacaccagtgtctcctagtatctgggtaataacctcctttcagtcttagtccacaccacacactaccctccagtctctcctactctttactgtcacagaaaagactctcagcttttattcacacctgccttcagaaggccaaaccattttgtgcctgaaaactgttacccactcgccccacactttacataagtatcacatatgttctttctacaaattggtatacaggtgccatttaatccattcaaatttggaagctacatcttcaagggtctgagagagctcactccccccatatattccccctttacatgttttcttataagacatacagtttaatcaattaacaaactaaacagcttatatactggcaatatattacagatgggtttatgtcagagtaatagatcacatgaaatggaccatgtggtaccccagtgcattatgtcttggtagagccctgaggacactgacagtagcatctctaagtaagtagtgctgtatgaatacagacacatgcggatctgtatctacatccatctgactaggccaaggagcaggtagatgcaagatagagacacacacatgctggatggggccactgcacaccttgtcatgccatttaaaagggcagttacaggttgccggttttgcagccattaaaattacactttatggaaaaggcttctctaattgtgtctgatttgctttctgtagtaagcatcattggaagaagaccaaagcaagagcaactagaagttaaatatacatttgagcttagctgcaatacagaaccctggggaagaagcaggctgaaagatttatttaattttaggcttggattctctcccttgctgttttcttgatgttgtgtgtctgcatttgtgtgtgtgtgtgtgtctgcgtgtgtgtgtgttccatcacatcatctcctgaagaacgctgggtttcgcaggcaggcggctagtcacctgcaacaacccaggggtcctgccgaggcttccaggctgctgtcagtgtcagatgccagggtctggtcggtggacatggaggagatgtcattgacagacgaggatggagggagactctcactgctgttcactgctgcacctgaaggagaaggctgtccttttactacaccatttttagtcttttcttctgaattcattacttccttgtagataagttctttccattcttcaattgtgtgttctctttcatccaactgcttgtcatatatctgaggtggaggcgcctccacttcggctgggtcataccagacgttgatgtagggatgctgtaaggcgtcgtccactgatattctttttgctgggtcaatcactagcatctttgacaacaagtccctggcttggctggctttgagtttattgtgctcggagtccgctgggaagagggaatctgggaagagtttggggaaggtgagtcccgcatacttgggccgattctccacatagtttcttactgtgggttgcaatttcttcatgaattctggacatggtgttcctagttgttcaattaccttattccactggtcaatatagtcccttcctggaaagaggattttgtggcgaaccatttctcccataatgcatcccacagaccatatatccacgttctccttgtagcccatccccaggatgacctcaggggctctgtaataacgtgtcaccacatatggagtcatcatgaagcttgtgcctgctgtcctggccagtccaaagtccaggattttcaatgtgcaatcagacttgactacaatgttacttggttttaaatccctgtgaataattccagcagaatggaggtgcttaatgccacacaacatttggtacagcaggtaagacattcgctcatggtctaattccatctgaatcacttgacataagttggcatccatcagttccattactaagtaaacatcttggaactcctccagcgttttctggggtgtgaagacatttaataaactaataatgtttttatggttcacacacttcatgaggaccagctcccggtacgctctcttggcatgtgtttggttctgaaagggtctgctgagcttcttaatggccacatttctgtcaaggacagcatcatacgcggcacaaactatgccctgagccccagagccaataggctttagattctggtagcgcttgagaactgtgaaggttgagtctcccacttccacactgtagaactggttgtcaactttgcttttgctcatgttgtaatgtttggcaatatatgacacatccacttgtttatcgaatccctgacaaaaggcaattttcacatccaatgttggttcactgcagtagtataagaaatggaggctcataaataccacagcttgtatggtttctcatctataggaaacgggtctaattcaacagtttcttgcataagttgccatagtgaagatctgagatgggcctgctgttggtgtttctcacactagcctggagctgagtcaatttagagagctgcgtgaaatacaggggtagaggaagcagcggcaaaatccctctgggctcgctgggtcccctgccacgccatttctgcctggcctcacaggggtccttgaggagggctgctggaggcactgggaaaggcatttttcactctcctcctcactccctagggtcatagttttgattctgaagttagaagtgtgggggtcgtcggctgcattttcaacttggcctaaaagttggagttcaccacactgcaggcgctaggaactctgccgctcggtcaccaacctgagcctctggctagtccgaagaacgcgaaaagccaggcccaaggcactggttgtcatggcaaccggggcgctggtctccctggcgacctcgtccctagggaggaggtggagctggatgccaggcgggccaatgaggtcgaggggagctcggggtgggagatctgcggtcctcccagtgccggggaatggttgagtgacaggaccgggggggcggagccggcgcggctgcccgaggtggagccccagtggtgcgagtagctccagcggccacgctgaggcgagggtgacacaccatgctcacggcccctggagaccgtcgtgctggcgagccgtgctccgtagctccccggtccgcctcggcagcggtcagagtcgcctacaggagttgagccgcccgcgccagaaggttttggcgaagctcttggagaggcgtcgagcacagtagggcggcgggggtgcgttgagcgctcgggggtcaggcagtcggccgggatcgccgctggggagcgtttccgaggcgaggaggaggaggaggagatgctgctcctcttctccccctcccc

SEQ ID NO: 9185 - RNA, 4295 nt, Homo sapiens
  source 1..4295: mol_type = other RNA
agacagtagttcttgcctggtttactctgagggggaaattcaccacttatgcaggtacgagagatagcctgtcaagcactttgaagatgctggctggagacttccttctgtcttgtgatgtcatcttgcggctgatgaaattccccttgagactctctttaaagcagcttcctgctctccgcacttaatcccatgtggtataaagtaagggaggggagaagccacagatatatcaagagaaaagtaccgagaaagaaaatcagtaaagaattagagatacagagaggagaagtttttaaaaaaaaaaaaaaaaaacaggaatatgaaagagagggagctcaagtgactgaggaggcatttttaacaatcaggttatctgcaatattaaccagaaaaaaaatggtagcaaaatagagaaaatgggccatttttattccaggggacaagctgcacaaaggaatgttcttctatttattttaaacaaatgactgcgtgtactgaatctgactgtgtgaaataatctcagaatggcagcaccactggcatggcgatggtgcaggtgggtgcagttccctgtggtctctattgcttgaagagagaaagaaagttccctattattatatttaaggcagttttcagagcactggcattcttgtttgctctgttttggggatattctatttgccaatcagttcacactcatcaaccatccacttcctgtctttcacttcttcaggtgaaatatcaccactctagtgagcaccaacatggtcagagtgcaaataactgtgatggatacttcgaagtgaataagaagggaagcctgattattgctgagatcaccttggtattgccttgtacataaccaagatgtttcacagtgcctccttaagtgctcaggaaagcactttcatttaatttaatttaagctaaattctggagattttgctaaacattgacattaatgcttcatggcttttaagacaaactcatattgctaaaactatttggcagcagtaaatttatgggcagagttattgctcttacatctactgcagtacaaaactcagatgatcagcccttcgattgctcatacttattaaaataaataaataaacatgaaacatcagccacattaaggagtcagggaaactcctgaggaataacaatgtctctggagatgttttcaaatgctaacctgagactcacactgtggtttgggggtttcattattattattattattttatttcagaagaggaaagtaatattatttctcaaaataaaactttggcagagtatgaatcagggaagcagcccacacatggaaaacacaatccacaatctgaaagtagtctaggcaggctcatttttttgttgaaggaattcacatggaggcaattctgctcagttccagagagagattcttatcatcaaaagcacacacaataaccttgcttcaccacctgccactttctccagtggcctcttgttgtgaccagtaattgagaaatgacaaatgggtatagagccaaatctctaaaacagggacaccagtgtctcctagtatctgggtaataacctcctttcagtcttagtccacaccacacactaccctccagtctctcctactctttactgtcacagaaaagactctcagcttttattcacacctgccttcagaaggccaaaccattttgtgcctgaaaactgttacccactcgccccacactttacataagtatcacatatgttctttctacaaattggtatacaggtgccatttaatccattcaaatttggaagctacatcttcaagggtctgagagagctcactccccccatatattccccctttacatgttttcttataagacatacagtttaatcaattaacaaactaaacagcttatatactggcaatatattacagatgggtttatgtcagagtaatagatcacatgaaatggaccatgtggtaccccagtgcattatgtcttggtagagccctgaggacactgacagtagcatctctaagtaagtagtgctgtatgaatacagacacatgcggatctgtatctacatccatctgactaggccaaggagcaggtagatgcaagatagagacacacacatgctggatggggccactgcacaccttgtcatgccatttaaaagggcagttacaggttgccggttttgcagccattaaaattacactttatggaaaaggcttctctaattgtgtctgatttgctttctgtagtaagcatcattggaagaagaccaaagcaagagcaactagaagttaaatatacatttgagcttagctgcaatacagaaccctggggaagaagcaggctgaaagatttatttaattttaggcttggattctctcccttgctgttttcttgatgttgtgtgtctgcatttgtgtgtgtgtgtgtgtctgcgtgtgtgtgtgttccatcacatcatctcctgaagaacgctgggtttcgcaggcaggcggctagtcacctgcaacaacccaggggtcctgccgaggcttccaggctgctgtcagtgtcagatgccagggtctggtcggtggacatggaggagatgtcattgacagacgaggatggagggagactctcactgctgttcactgctgcacctgaaggagaaggctgtccttttactacaccatttttagtcttttcttctgaattcattacttccttgtagataagttctttccattcttcaattgtgtgttctctttcatccaactgcttgtcatatatctgaggtggaggcgcctccacttcggctgggtcataccagacgttgatgtagggatgctgtaaggcgtcgtccactgatattctttttgctgggtcaatcactagcatctttgacaacaagtccctggcttggctggctttgagtttattgtgctcggagtccgctgggaagagggaatctgggaagagtttggggaaggtgagtcccgcatacttgggccgattctccacatagtttcttactgtgggttgcaatttcttcatgaattctggacatggtgttcctagttgttcaattaccttattccactggtcaatatagtcccttcctggaaagaggattttgtggcgaaccatttctcccataatgcatcccacagaccatatatccacgttctccttgtagcccatccccaggatgacctcaggggctctgtaataacgtgtcaccacatatggagtcatcatgaagcttgtgcctgctgtcctggccagtccaaagtccaggattttcaatgtgcaatcagacttgactacaatgttacttggttttaaatccctgtgaataattccagcagaatggaggtgcttaatgccacacaacatttggtacagcaggtaagacattcgctcatggtctaattccatctgaatcacttgacataagttggcatccatcagttccattactaagtaaacatcttggaactcctccagcgttttctggggtgtgaagacatttaataaactaataatgtttttatggttcacacacttcatgaggaccagctcccggtacgctctcttggcatgtgtttggttctgaaagggtctgctgagcttcttaatggccacatttctgtcaaggacagcatcatacgcggcacaaactatgccctgagccccagagccaataggctttagattctggtagcgcttgagaactgtgaaggttgagtctcccacttccacactgtagaactggttgtcaactttgcttttgctcatgttgtaatgtttggcaatatatgacacatccacttgtttatcgaatccctgacaaaaggcaattttcacatccaatgttggttcactgcagtagtataagaaatggaggctcataaataccacagcttgtatggtttctcatctataggaaacgggtctaattcaacagtttcttgcataagttgccatagtgaagatctgagatgggcctgctgttggtgtttctcacactagccttgggaagaagcatagtcaaataaaaatggaaaccttagtctcagttccactgtgactatgactacccatcagatgttgggcagatagtggctctgtcgacatgtttcttcatctacaatgtatcaggtctagatcacatgataattatggttcttttaccgtgacttcatttatctgggcaatctccacaaatctagaaagtagctttgatgttttcatcagacattattcatttataaactttagagtgccatctgtgtg

SEQ ID NO: 9186 - RNA, 4197 nt, Homo sapiens
  source 1..4197: mol_type = other RNA
agacagtagttcttgcctggtttactctgagggggaaattcaccacttatgcaggtacgagagatagcctgtcaagcactttgaagatgctggctggagacttccttctgtcttgtgatgtcatcttgcggctgatgaaattccccttgagactctctttaaagcagcttcctgctctccgcacttaatcccatgtggtataaagtaagggaggggagaagccacagatatatcaagagaaaagtaccgagaaagaaaatcagtaaagaattagagatacagagaggagaagtttttaaaaaaaaaaaaaaaaaacaggaatatgaaagagagggagctcaagtgactgaggaggcatttttaacaatcaggttatctgcaatattaaccagaaaaaaaatggtagcaaaatagagaaaatgggccatttttattccaggggacaagctgcacaaaggaatgttcttctatttattttaaacaaatgactgcgtgtactgaatctgactgtgtgaaataatctcagaatggcagcaccactggcatggcgatggtgcaggtgggtgcagttccctgtggtctctattgcttgaagagagaaagaaagttccctattattatatttaaggcagttttcagagcactggcattcttgtttgctctgttttggggatattctatttgccaatcagttcacactcatcaaccatccacttcctgtctttcacttcttcaggtgaaatatcaccactctagtgagcaccaacatggtcagagtgcaaataactgtgatggatacttcgaagtgaataagaagggaagcctgattattgctgagatcaccttggtattgccttgtacataaccaagatgtttcacagtgcctccttaagtgctcaggaaagcactttcatttaatttaatttaagctaaattctggagattttgctaaacattgacattaatgcttcatggcttttaagacaaactcatattgctaaaactatttggcagcagtaaatttatgggcagagttattgctcttacatctactgcagtacaaaactcagatgatcagcccttcgattgctcatacttattaaaataaataaataaacatgaaacatcagccacattaaggagtcagggaaactcctgaggaataacaatgtctctggagatgttttcaaatgctaacctgagactcacactgtggtttgggggtttcattattattattattattttatttcagaagaggaaagtaatattatttctcaaaataaaactttggcagagtatgaatcagggaagcagcccacacatggaaaacacaatccacaatctgaaagtagtctaggcaggctcatttttttgttgaaggaattcacatggaggcaattctgctcagttccagagagagattcttatcatcaaaagcacacacaataaccttgcttcaccacctgccactttctccagtggcctcttgttgtgaccagtaattgagaaatgacaaatgggtatagagccaaatctctaaaacagggacaccagtgtctcctagtatctgggtaataacctcctttcagtcttagtccacaccacacactaccctccagtctctcctactctttactgtcacagaaaagactctcagcttttattcacacctgccttcagaaggccaaaccattttgtgcctgaaaactgttacccactcgccccacactttacataagtatcacatatgttctttctacaaattggtatacaggtgccatttaatccattcaaatttggaagctacatcttcaagggtctgagagagctcactccccccatatattccccctttacatgttttcttataagacatacagtttaatcaattaacaaactaaacagcttatatactggcaatatattacagatgggtttatgtcagagtaatagatcacatgaaatggaccatgtggtaccccagtgcattatgtcttggtagagccctgaggacactgacagtagcatctctaagtaagtagtgctgtatgaatacagacacatgcggatctgtatctacatccatctgactaggccaaggagcaggtagatgcaagatagagacacacacatgctggatggggccactgcacaccttgtcatgccatttaaaagggcagttacaggttgccggttttgcagccattaaaattacactttatggaaaaggcttctctaattgtgtctgatttgctttctgtagtaagcatcattggaagaagaccaaagcaagagcaactagaagttaaatatacatttgagcttagctgcaatacagaaccctggggaagaagcaggctgaaagatttatttaattttaggcttggattctctcccttgctgttttcttgatgttgtgtgtctgcatttgtgtgtgtgtgtgtgtctgcgtgtgtgtgtgttccatcacatcatctcctgaagaacgctgggtttcgcaggcaggcggctagtcacctgcaacaacccaggggtcctgccgaggcttccaggctgctgtcagtgtcagatgccagggtctggtcggtggacatggaggagatgtcattgacagacgaggatggagggagactctcactgctgttcactgctgcacctgaaggagaaggctgtccttttactacaccatttttagtcttttcttctgaattcattacttccttgtagataagttctttccattcttcaattgtgtgttctctttcatccaactgcttgtcatatatctgaggtggaggcgcctccacttcggctgggtcataccagacgttgatgtagggatgctgtaaggcgtcgtccactgatattctttttgctgggtcaatcactagcatctttgacaacaagtccctggcttggctggctttgagtttattgtgctcggagtccgctgggaagagggaatctgggaagagtttggggaaggtgagtcccgcatacttgggccgattctccacatagtttcttactgtgggttgcaatttcttcatgaattctggacatggtgttcctagttgttcaattaccttattccactggtcaatatagtcccttcctggaaagaggattttgtggcgaaccatttctcccataatgcatcccacagaccatatatccacgttctccttgtagcccatccccaggatgacctcaggggctctgtaataacgtgtcaccacatatggagtcatcatgaagcttgtgcctgctgtcctggccagtccaaagtccaggattttcaatgtgcaatcagacttgactacaatgttacttggttttaaatccctgtgaataattccagcagaatggaggtgcttaatgccacacaacatttggtacagcaggtaagacattcgctcatggtctaattccatctgaatcacttgacataagttggcatccatcagttccattactaagtaaacatcttggaactcctccagcgttttctggggtgtgaagacatttaataaactaataatgtttttatggttcacacacttcatgaggaccagctcccggtacgctctcttggcatgtgtttggttctgaaagggtctgctgagcttcttaatggccacatttctgtcaaggacagcatcatacgcggcacaaactatgccctgagccccagagccaataggctttagattctggtagcgcttgagaactgtgaaggttgagtctcccacttccacactgtagaactggttgtcaactttgcttttgctcatgttgtaatgtttggcaatatatgacacatccacttgtttatcgaatccctgacaaaaggcaattttcacatccaatgttggttcactgcagtagtataagaaatggaggctcataaataccacagcttgtatggtttctcatctataggaaacgggtctaattcaacagtttcttgcataagttgccatagtgaagatctgagatgggcctgctgttggtgtttctcacactagcgcatttttcactctcctcctcactccctagggtcatagttttgattctgaagttagaagtgtgggggtcgtcggctgcattttcaacttggcctaaaagttggagttcaccacactgcaggcgctaggaactctgccgctcggtcaccaacctgagcctctggct

SEQ ID NO: 9187 - RNA, 6939 nt, Homo sapiens
  source 1..6939: mol_type = other RNA
agacagtagttcttgcctggtttactctgagggggaaattcaccacttatgcaggtacgagagatagcctgtcaagcactttgaagatgctggctggagacttccttctgtcttgtgatgtcatcttgcggctgatgaaattccccttgagactctctttaaagcagcttcctgctctccgcacttaatcccatgtggtataaagtaagggaggggagaagccacagatatatcaagagaaaagtaccgagaaagaaaatcagtaaagaattagagatacagagaggagaagtttttaaaaaaaaaaaaaaaaaacaggaatatgaaagagagggagctcaagtgactgaggaggcatttttaacaatcaggttatctgcaatattaaccagaaaaaaaatggtagcaaaatagagaaaatgggccatttttattccaggggacaagctgcacaaaggaatgttcttctatttattttaaacaaatgactgcgtgtactgaatctgactgtgtgaaataatctcagaatggcagcaccactggcatggcgatggtgcaggtgggtgcagttccctgtggtctctattgcttgaagagagaaagaaagttccctattattatatttaaggcagttttcagagcactggcattcttgtttgctctgttttggggatattctatttgccaatcagttcacactcatcaaccatccacttcctgtctttcacttcttcaggtgaaatatcaccactctagtgagcaccaacatggtcagagtgcaaataactgtgatggatacttcgaagtgaataagaagggaagcctgattattgctgagatcaccttggtattgccttgtacataaccaagatgtttcacagtgcctccttaagtgctcaggaaagcactttcatttaatttaatttaagctaaattctggagattttgctaaacattgacattaatgcttcatggcttttaagacaaactcatattgctaaaactatttggcagcagtaaatttatgggcagagttattgctcttacatctactgcagtacaaaactcagatgatcagcccttcgattgctcatacttattaaaataaataaataaacatgaaacatcagccacattaaggagtcagggaaactcctgaggaataacaatgtctctggagatgttttcaaatgctaacctgagactcacactgtggtttgggggtttcattattattattattattttatttcagaagaggaaagtaatattatttctcaaaataaaactttggcagagtatgaatcagggaagcagcccacacatggaaaacacaatccacaatctgaaagtagtctaggcaggctcatttttttgttgaaggaattcacatggaggcaattctgctcagttccagagagagattcttatcatcaaaagcacacacaataaccttgcttcaccacctgccactttctccagtggcctcttgttgtgaccagtaattgagaaatgacaaatgggtatagagccaaatctctaaaacagggacaccagtgtctcctagtatctgggtaataacctcctttcagtcttagtccacaccacacactaccctccagtctctcctactctttactgtcacagaaaagactctcagcttttattcacacctgccttcagaaggccaaaccattttgtgcctgaaaactgttacccactcgccccacactttacataagtatcacatatgttctttctacaaattggtatacaggtgccatttaatccattcaaatttggaagctacatcttcaagggtctgagagagctcactccccccatatattccccctttacatgttttcttataagacatacagtttaatcaattaacaaactaaacagcttatatactggcaatatattacagatgggtttatgtcagagtaatagatcacatgaaatggaccatgtggtaccccagtgcattatgtcttggtagagccctgaggacactgacagtagcatctctaagtaagtagtgctgtatgaatacagacacatgcggatctgtatctacatccatctgactaggccaaggagcaggtagatgcaagatagagacacacacatgctggatggggccactgcacaccttgtcatgccatttaaaagggcagttacaggttgccggttttgcagccattaaaattacactttatggaaaaggcttctctaattgtgtctgatttgctttctgtagtaagcatcattggaagaagaccaaagcaagagcaactagaagttaaatatacatttgagcttagctgcaatacagaaccctggggaagaagcaggctgaaagatttatttaattttaggcttggattctctcccttgctgttttcttgatgttgtgtgtctgcatttgtgtgtgtgtgtgtgtctgcgtgtgtgtgtgttccatcacatcatctcctgaagaacgctgggtttcgcaggcaggcggctagtcacctgcaacaacccaggggtcctgccgaggcttccaggctgctgtcagtgtcagatgccagggtctggtcggtggacatggaggagatgtcattgacagacgaggatggagggagactctcactgctgttcactgctgcacctgaaggagaaggctgtccttttactacaccatttttagtcttttcttctgaattcattacttccttgtagataagttctttccattcttcaattgtgtgttctctttcatccaactgcttgtcatatatctgaggtggaggcgcctccacttcggctgggtcataccagacgttgatgtagggatgctgtaaggcgtcgtccactgatattctttttgctgggtcaatcactagcatctttgacaacaagtccctggcttggctggctttgagtttattgtgctcggagtccgctgggaagagggaatctgggaagagtttggggaaggtgagtcccgcatacttgggccgattctccacatagtttcttactgtgggttgcaatttcttcatgaattctggacatggtgttcctagttgttcaattaccttattccactggtcaatatagtcccttcctggaaagaggattttgtggcgaaccatttctcccataatgcatcccacagaccatatatccacgttctccttgtagcccatccccaggatgacctcaggggctctgtaataacgtgtcaccacatatggagtcatcatgaagcttgtgcctgctgtcctggccagtccaaagtccaggattttcaatgtgcaatcagacttgactacaatgttacttggttttaaatccctgtgaataattccagcagaatggaggtgcttaatgccacacaacatttggtacagcaggtaagacattcgctcatggtctaattccatctgaatcacttgacataagttggcatccatcagttccattactaagtaaacatcttggaactcctccagcgttttctggggtgtgaagacatttaataaactaataatgtttttatggttcacacacttcatgaggaccagctcccggtacgctctcttggcatgtgtttggttctgaaagggtctgctgagcttcttaatggccacatttctgtcaaggacagcatcatacgcggcacaaactatgccctgagccccagagccaataggctttagattctggtagcgcttgagaactgtgaaggttgagtctcccacttccacactgtagaactggttgtcaactttgcttttgctcatgttgtaatgtttggcaatatatgacacatccacttgtttatcgaatccctgacaaaaggcaattttcacatccaatgttggttcactgcagtagtataagaaatggaggctcataaatacttgtctctgagcctcttctctctcctctccaaccagaaatatgttggatcctgctcataccagctctctagcaccaattgtgaccatcttttttttttttttagacaaagtctggctctgtcgccaggctggagtgcagtggtgcaatcttggctcacagcaacctccgactccctggttgaagcaaaaagtgcaaaaagtgtctacaaaagcatttaattttgccttttgctccctgctgcctaatggcttctctcctacttccctattacccactggggggaagaaaaaggaaataagggtttatagacatcatctgtggcatatcctgggaaagaaactgagttctttttatttttatgatttctaatatattaatgttaaaattaaaatccagggctccagtgttccatgttagctcttagcagtgataatctaataaaataatttaaaagctaatataacaagcttaaatttgatgcttggattactttttaaagtgcctaagtattgagataaaaactaatgcttatgtgactagatggttaagcagacagtaactttttttaagtgttaagttatatttgcaagcaaagttacacagagtaagatgcttaataaccagtgttacttgtttctagttgataaatctaaaagcattgccaggatggtggcacatcaaacattggcttattatgagtatgtaattgtattattttcctacctttagccacatctccactatcaaccatctaaatttaattttgttaacaaacggtttaccaaacattaacaatctatgctatctgttgaaggcttggagtagatgttaccatttatttcaaagaaaaaacaagcacacacaaacatggaatactactcctaaggatgcaaaaaattaaggagaaattttagatatatatcacaaagtataacatcatgatgtttttaaatatgtacctcagttataagtaaaacatacaaaagaggatgggcttacacagggacaattgctaaagggttttctataacaatactttgtctacatcactattttggcatgttttactcatatcaaaagacagacgtacaatcttaaatatccaagattgtttcacataaaacctaggctaatagccaaattggtctgaagttcttactaacaaatgtagctttcaaaaacaacaaaagaaatggcctggatacccatcaagtagacagaatttattctaattcactaactccctagtgtcctagtacattttgtattagaataaggattgcctttggctatggagtctactccaaaatatgaacatagtggagcaatcatcttccacttagcttattatacatcacagggaacgttagttatgtgtagtttaaggaaatatgttctgaatcacagtaagtgactgaaaggcaaaaggagttatgtctagttcagggatctatatgagttgaaggttctgaaatacagcaaaacccgctagtaaaaaaaatgaataaaatttactaaatattggaagtgttaaatcaactgaagtttcaaacagaagcattaacctagcaattttttaaaaactaaaaataaattactaaaaaataaacatatagtcaccttaactgagtgatcaatgttaacatcactagtaatatgacatatcaatgttatgtactccctgatagaatacacaggaaaaagtccttcccccaaattcataacctcaatcaatcataagaaaacattaagacaagtccaaatggaaggatgatttacaaactacctgaacaaatgttaaaagtcacaagagacaaagaaagacaaaggatttatcacagattggaggggattaaggacatggtaagtaaacacaatgtgggattctggatcaaatcttgaaagagagagaggacattggtgggaaaactggggaaatatgttaaagttcatcatttgttaatagtaatgtctcaatgttcatttcttttttttggcttttcatggttatgtaaagtgttaacctttggggaagctgggtgaagaccatgtatgggaactgttcatattatctttgtaaattttatgtaagtctaatattatgacaaaattaagttttgaaagtacataaatttatagtatatggagaaaaacagaaatgtgcacagtttatcattatacaaaacacacatttgatggccgtcttattgatttgttgttttctctttgatatcttgttttcttttcttttttatcttctaagcctctgatcacttatcttagtcaaggttgagcagatagagaagtacgcacatcctgtagcctgaaagcctagcttcagattctatttctaccacttactgtgtgatgtggggcaattaaattaactttcagtgcccagtttctttatggtacaaacaggaagaataatatctgccacatagagctgttgtaaaaataaatgagttaatatatgcaaagcatatggtagagcagtgtgtgcccagagtgagtaccatttgacagaaacaccagaatagttgaagacagagtactgtcttttacttcagaaacaaagtgggacagctgtttctctccctttgctctcttgctgcaatgaagctgacattactagggggggctcaactaaccaaacactcccaattggaatttcgattcctgaaaggataatgagtgaaggggcaaattagcagaatcaaggaagcagaaaattcctcactccagcattctagccacactccccgcaagtggaaatcaggctgtgagcttctctgactacgttgtttcccgcccatcttccaaccctggatctccagtgctcctgcagctctgtgagccatcatatgctcttccaacaaatctctttattccttaaattaaaaaattaactcaaaatggattaaagacttaaatgtaagatttcaaactataaaaaccctagaagaaaacctaggaaatacctttcttgacatcagccttagcaaacaatttgtggctaag

SEQ ID NO: 9188 - RNA, 4445 nt, Homo sapiens
  source 1..4445: mol_type = other RNA
agacagtagttcttgcctggtttactctgagggggaaattcaccacttatgcaggtacgagagatagcctgtcaagcactttgaagatgctggctggagacttccttctgtcttgtgatgtcatcttgcggctgatgaaattccccttgagactctctttaaagcagcttcctgctctccgcacttaatcccatgtggtataaagtaagggaggggagaagccacagatatatcaagagaaaagtaccgagaaagaaaatcagtaaagaattagagatacagagaggagaagtttttaaaaaaaaaaaaaaaaaacaggaatatgaaagagagggagctcaagtgactgaggaggcatttttaacaatcaggttatctgcaatattaaccagaaaaaaaatggtagcaaaatagagaaaatgggccatttttattccaggggacaagctgcacaaaggaatgttcttctatttattttaaacaaatgactgcgtgtactgaatctgactgtgtgaaataatctcagaatggcagcaccactggcatggcgatggtgcaggtgggtgcagttccctgtggtctctattgcttgaagagagaaagaaagttccctattattatatttaaggcagttttcagagcactggcattcttgtttgctctgttttggggatattctatttgccaatcagttcacactcatcaaccatccacttcctgtctttcacttcttcaggtgaaatatcaccactctagtgagcaccaacatggtcagagtgcaaataactgtgatggatacttcgaagtgaataagaagggaagcctgattattgctgagatcaccttggtattgccttgtacataaccaagatgtttcacagtgcctccttaagtgctcaggaaagcactttcatttaatttaatttaagctaaattctggagattttgctaaacattgacattaatgcttcatggcttttaagacaaactcatattgctaaaactatttggcagcagtaaatttatgggcagagttattgctcttacatctactgcagtacaaaactcagatgatcagcccttcgattgctcatacttattaaaataaataaataaacatgaaacatcagccacattaaggagtcagggaaactcctgaggaataacaatgtctctggagatgttttcaaatgctaacctgagactcacactgtggtttgggggtttcattattattattattattttatttcagaagaggaaagtaatattatttctcaaaataaaactttggcagagtatgaatcagggaagcagcccacacatggaaaacacaatccacaatctgaaagtagtctaggcaggctcatttttttgttgaaggaattcacatggaggcaattctgctcagttccagagagagattcttatcatcaaaagcacacacaataaccttgcttcaccacctgccactttctccagtggcctcttgttgtgaccagtaattgagaaatgacaaatgggtatagagccaaatctctaaaacagggacaccagtgtctcctagtatctgggtaataacctcctttcagtcttagtccacaccacacactaccctccagtctctcctactctttactgtcacagaaaagactctcagcttttattcacacctgccttcagaaggccaaaccattttgtgcctgaaaactgttacccactcgccccacactttacataagtatcacatatgttctttctacaaattggtatacaggtgccatttaatccattcaaatttggaagctacatcttcaagggtctgagagagctcactccccccatatattccccctttacatgttttcttataagacatacagtttaatcaattaacaaactaaacagcttatatactggcaatatattacagatgggtttatgtcagagtaatagatcacatgaaatggaccatgtggtaccccagtgcattatgtcttggtagagccctgaggacactgacagtagcatctctaagtaagtagtgctgtatgaatacagacacatgcggatctgtatctacatccatctgactaggccaaggagcaggtagatgcaagatagagacacacacatgctggatggggccactgcacaccttgtcatgccatttaaaagggcagttacaggttgccggttttgcagccattaaaattacactttatggaaaaggcttctctaattgtgtctgatttgctttctgtagtaagcatcattggaagaagaccaaagcaagagcaactagaagttaaatatacatttgagcttagctgcaatacagaaccctggggaagaagcaggctgaaagatttatttaattttaggcttggattctctcccttgctgttttcttgatgttgtgtgtctgcatttgtgtgtgtgtgtgtgtctgcgtgtgtgtgtgttccatcacatcatctcctgaagaacgctgggtttcgcaggcaggcggctagtcacctgcaacaacccaggggtcctgccgaggcttccaggctgctgtcagtgtcagatgccagggtctggtcggtggacatggaggagatgtcattgacagacgaggatggagggagactctcactgctgttcactgctgcacctgaaggagaaggctgtccttttactacaccatttttagtcttttcttctgaattcattacttccttgtagataagttctttccattcttcaattgtgtgttctctttcatccaactgcttgtcatatatctgaggtggaggcgcctccacttcggctgggtcataccagacgttgatgtagggatgctgtaaggcgtcgtccactgatattctttttgctgggtcaatcactagcatctttgacaacaagtccctggcttggctggctttgagtttattgtgctcggagtccgctgggaagagggaatctgggaagagtttggggaaggtgagtcccgcatacttgggccgattctccacatagtttcttactgtgggttgcaatttcttcatgaattctggacatggtgttcctagttgttcaattaccttattccactggtcaatatagtcccttcctggaaagaggattttgtggcgaaccatttctcccataatgcatcccacagaccatatatccacgttctccttgtagcccatccccaggatgacctcaggggctctgtaataacgtgtcaccacatatggagtcatcatgaagcttgtgcctgctgtcctggccagtccaaagtccaggattttcaatgtgcaatcagacttgactacaatgttacttggttttaaatccctgtgaataattccagcagaatggaggtgcttaatgccacacaacatttggtacagcaggtaagacattcgctcatggtctaattccatctgaatcacttgacataagttggcatccatcagttccattactaagtaaacatcttggaactcctccagcgttttctggggtgtgaagacatttaataaactaataatgtttttatggttcacacacttcatgaggaccagctcccggtacgctctcttggcatgtgtttggttctgaaagggtctgctgagcttcttaatggccacatttctgtcaaggacagcatcatacgcggcacaaactatgccctgagccccagagccaataggctttagattctggtagcgcttgagaactgtgaaggttgagtctcccacttccacactgtagaactggttgtcaactttgcttttgctcatgttgtaatgtttggcaatatatgacacatccacttgtttatcgaatccctgtaaggaacacacacctgacaaaaggcaattttcacatccaatgttggttcactgcagtagtataagaaatggaggctcataaataccacagcttgtatggtttctcatctataggaaacgggtctaattcaacagtttcttgcataagttgccatagtgaagatctgagatgggcctgctgttggtgtttctcacactagccattccgtgcctgagaactacgatcctgatccggcagtgtttgccccagaaatcctccctacttgtttttcattaaccacattccagactaacatggaagagattctttggagatatggagattgtttaaaattaacgatggacaggtgatttccaagaaaacccaatcttaaactcactcaagcccctaggaattgaggggtgaggacaaaaaaggaaatttgtaaaaatgaaaaaagaaaagaaaaaggtaagcatatagcaagcaccacccacccccataaaaataaaaagtgaaggggaggttaaagaaaatagaagaagagtggcttgctgaatcaccctctttcactgcctggaaaccattgtgcagcgtgatgctgcctgtaccattgt

SEQ ID NO: 9189 - RNA, 4126 nt, Homo sapiens
  source 1..4126: mol_type = other RNA
agacagtagttcttgcctggtttactctgagggggaaattcaccacttatgcaggtacgagagatagcctgtcaagcactttgaagatgctggctggagacttccttctgtcttgtgatgtcatcttgcggctgatgaaattccccttgagactctctttaaagcagcttcctgctctccgcacttaatcccatgtggtataaagtaagggaggggagaagccacagatatatcaagagaaaagtaccgagaaagaaaatcagtaaagaattagagatacagagaggagaagtttttaaaaaaaaaaaaaaaaaacaggaatatgaaagagagggagctcaagtgactgaggaggcatttttaacaatcaggttatctgcaatattaaccagaaaaaaaatggtagcaaaatagagaaaatgggccatttttattccaggggacaagctgcacaaaggaatgttcttctatttattttaaacaaatgactgcgtgtactgaatctgactgtgtgaaataatctcagaatggcagcaccactggcatggcgatggtgcaggtgggtgcagttccctgtggtctctattgcttgaagagagaaagaaagttccctattattatatttaaggcagttttcagagcactggcattcttgtttgctctgttttggggatattctatttgccaatcagttcacactcatcaaccatccacttcctgtctttcacttcttcaggtgaaatatcaccactctagtgagcaccaacatggtcagagtgcaaataactgtgatggatacttcgaagtgaataagaagggaagcctgattattgctgagatcaccttggtattgccttgtacataaccaagatgtttcacagtgcctccttaagtgctcaggaaagcactttcatttaatttaatttaagctaaattctggagattttgctaaacattgacattaatgcttcatggcttttaagacaaactcatattgctaaaactatttggcagcagtaaatttatgggcagagttattgctcttacatctactgcagtacaaaactcagatgatcagcccttcgattgctcatacttattaaaataaataaataaacatgaaacatcagccacattaaggagtcagggaaactcctgaggaataacaatgtctctggagatgttttcaaatgctaacctgagactcacactgtggtttgggggtttcattattattattattattttatttcagaagaggaaagtaatattatttctcaaaataaaactttggcagagtatgaatcagggaagcagcccacacatggaaaacacaatccacaatctgaaagtagtctaggcaggctcatttttttgttgaaggaattcacatggaggcaattctgctcagttccagagagagattcttatcatcaaaagcacacacaataaccttgcttcaccacctgccactttctccagtggcctcttgttgtgaccagtaattgagaaatgacaaatgggtatagagccaaatctctaaaacagggacaccagtgtctcctagtatctgggtaataacctcctttcagtcttagtccacaccacacactaccctccagtctctcctactctttactgtcacagaaaagactctcagcttttattcacacctgccttcagaaggccaaaccattttgtgcctgaaaactgttacccactcgccccacactttacataagtatcacatatgttctttctacaaattggtatacaggtgccatttaatccattcaaatttggaagctacatcttcaagggtctgagagagctcactccccccatatattccccctttacatgttttcttataagacatacagtttaatcaattaacaaactaaacagcttatatactggcaatatattacagatgggtttatgtcagagtaatagatcacatgaaatggaccatgtggtaccccagtgcattatgtcttggtagagccctgaggacactgacagtagcatctctaagtaagtagtgctgtatgaatacagacacatgcggatctgtatctacatccatctgactaggccaaggagcaggtagatgcaagatagagacacacacatgctggatggggccactgcacaccttgtcatgccatttaaaagggcagttacaggttgccggttttgcagccattaaaattacactttatggaaaaggcttctctaattgtgtctgatttgctttctgtagtaagcatcattggaagaagaccaaagcaagagcaactagaagttaaatatacatttgagcttagctgcaatacagaaccctggggaagaagcaggctgaaagatttatttaattttaggcttggattctctcccttgctgttttcttgatgttgtgtgtctgcatttgtgtgtgtgtgtgtgtctgcgtgtgtgtgtgttccatcacatcatctcctgaagaacgctgggtttcgcaggcaggcggctagtcacctgcaacaacccaggggtcctgccgaggcttccaggctgctgtcagtgtcagatgccagggtctggtcggtggacatggaggagatgtcattgacagacgaggatggagggagactctcactgctgttcactgctgcacctgaaggagaaggctgtccttttactacaccatttttagtcttttcttctgaattcattacttccttgtagataagttctttccattcttcaattgtgtgttctctttcatccaactgcttgtcatatatctgaggtggaggcgcctccacttcggctgggtcataccagacgttgatgtagggatgctgtaaggcgtcgtccactgatattctttttgctgggtcaatcactagcatctttgacaacaagtccctggcttggctggctttgagtttattgtgctcggagtccgctgggaagagggaatctgggaagagtttggggaaggtgagtcccgcatacttgggccgattctccacatagtttcttactgtgggttgcaatttcttcatgaattctggacatggtgttcctagttgttcaattaccttattccactggtcaatatagtcccttcctggaaagaggattttgtggcgaaccatttctcccataatgcatcccacagaccatatatccacgttctccttgtagcccatccccaggatgacctcaggggctctgtaataacgtgtcaccacatatggagtcatcatgaagcttgtgcctgctgtcctggccagtccaaagtccaggattttcaatgtgcaatcagacttgactacaatgttacttggttttaaatccctgtgaataattccagcagaatggaggtgcttaatgccacacaacatttggtacagcaggtaagacattcgctcatggtctaattccatctgaatcacttgacataagttggcatccatcagttccattactaagtaaacatcttggaactcctccagcgttttctggggtgtgaagacatttaataaactaataatgtttttatggttcacacacttcatgaggaccagctcccggtacgctctcttggcatgtgtttggttctgaaagggtctgctgagcttcttaatggccacatttctgtcaaggacagcatcatacgcggcacaaactatgccctgagccccagagccaataggctttagattctggtagcgcttgagaactgtgaaggttgagtctcccacttccacactgtagaactggttgtcaactttgcttttgctcatgttgtaatgtttggcaatatatgacacatccacttgtttatcgaatcccttgttttacctgtaaggaacacacacctgacaaaaggcaattttcacatccaatgttggttcactgcagtagtataagaaatggaggctcataaataccacagcttgtatggtttctcatctataggaaacgggtctaattcaacagtttcttgcataagttgccatagtgaagatctgagatgggcctgctgttggtgtttctcacactagccagacaatgacagcaaaaacacactcagcccctctgggatctgttcataaacatccccttccagcat

SEQ ID NO: 9190 - RNA, 4109 nt, Homo sapiens
  source 1..4109: mol_type = other RNA
agacagtagttcttgcctggtttactctgagggggaaattcaccacttatgcaggtacgagagatagcctgtcaagcactttgaagatgctggctggagacttccttctgtcttgtgatgtcatcttgcggctgatgaaattccccttgagactctctttaaagcagcttcctgctctccgcacttaatcccatgtggtataaagtaagggaggggagaagccacagatatatcaagagaaaagtaccgagaaagaaaatcagtaaagaattagagatacagagaggagaagtttttaaaaaaaaaaaaaaaaaacaggaatatgaaagagagggagctcaagtgactgaggaggcatttttaacaatcaggttatctgcaatattaaccagaaaaaaaatggtagcaaaatagagaaaatgggccatttttattccaggggacaagctgcacaaaggaatgttcttctatttattttaaacaaatgactgcgtgtactgaatctgactgtgtgaaataatctcagaatggcagcaccactggcatggcgatggtgcaggtgggtgcagttccctgtggtctctattgcttgaagagagaaagaaagttccctattattatatttaaggcagttttcagagcactggcattcttgtttgctctgttttggggatattctatttgccaatcagttcacactcatcaaccatccacttcctgtctttcacttcttcaggtgaaatatcaccactctagtgagcaccaacatggtcagagtgcaaataactgtgatggatacttcgaagtgaataagaagggaagcctgattattgctgagatcaccttggtattgccttgtacataaccaagatgtttcacagtgcctccttaagtgctcaggaaagcactttcatttaatttaatttaagctaaattctggagattttgctaaacattgacattaatgcttcatggcttttaagacaaactcatattgctaaaactatttggcagcagtaaatttatgggcagagttattgctcttacatctactgcagtacaaaactcagatgatcagcccttcgattgctcatacttattaaaataaataaataaacatgaaacatcagccacattaaggagtcagggaaactcctgaggaataacaatgtctctggagatgttttcaaatgctaacctgagactcacactgtggtttgggggtttcattattattattattattttatttcagaagaggaaagtaatattatttctcaaaataaaactttggcagagtatgaatcagggaagcagcccacacatggaaaacacaatccacaatctgaaagtagtctaggcaggctcatttttttgttgaaggaattcacatggaggcaattctgctcagttccagagagagattcttatcatcaaaagcacacacaataaccttgcttcaccacctgccactttctccagtggcctcttgttgtgaccagtaattgagaaatgacaaatgggtatagagccaaatctctaaaacagggacaccagtgtctcctagtatctgggtaataacctcctttcagtcttagtccacaccacacactaccctccagtctctcctactctttactgtcacagaaaagactctcagcttttattcacacctgccttcagaaggccaaaccattttgtgcctgaaaactgttacccactcgccccacactttacataagtatcacatatgttctttctacaaattggtatacaggtgccatttaatccattcaaatttggaagctacatcttcaagggtctgagagagctcactccccccatatattccccctttacatgttttcttataagacatacagtttaatcaattaacaaactaaacagcttatatactggcaatatattacagatgggtttatgtcagagtaatagatcacatgaaatggaccatgtggtaccccagtgcattatgtcttggtagagccctgaggacactgacagtagcatctctaagtaagtagtgctgtatgaatacagacacatgcggatctgtatctacatccatctgactaggccaaggagcaggtagatgcaagatagagacacacacatgctggatggggccactgcacaccttgtcatgccatttaaaagggcagttacaggttgccggttttgcagccattaaaattacactttatggaaaaggcttctctaattgtgtctgatttgctttctgtagtaagcatcattggaagaagaccaaagcaagagcaactagaagttaaatatacatttgagcttagctgcaatacagaaccctggggaagaagcaggctgaaagatttatttaattttaggcttggattctctcccttgctgttttcttgatgttgtgtgtctgcatttgtgtgtgtgtgtgtgtctgcgtgtgtgtgtgttccatcacatcatctcctgaagaacgctgggtttcgcaggcaggcggctagtcacctgcaacaacccaggggtcctgccgaggcttccaggctgctgtcagtgtcagatgccagggtctggtcggtggacatggaggagatgtcattgacagacgaggatggagggagactctcactgctgttcactgctgcacctgaaggagaaggctgtccttttactacaccatttttagtcttttcttctgaattcattacttccttgtagataagttctttccattcttcaattgtgtgttctctttcatccaactgcttgtcatatatctgaggtggaggcgcctccacttcggctgggtcataccagacgttgatgtagggatgctgtaaggcgtcgtccactgatattctttttgctgggtcaatcactagcatctttgacaacaagtccctggcttggctggctttgagtttattgtgctcggagtccgctgggaagagggaatctgggaagagtttggggaaggtgagtcccgcatacttgggccgattctccacatagtttcttactgtgggttgcaatttcttcatgaattctggacatggtgttcctagttgttcaattaccttattccactggtcaatatagtcccttcctggaaagaggattttgtggcgaaccatttctcccataatgcatcccacagaccatatatccacgttctccttgtagcccatccccaggatgacctcaggggctctgtaataacgtgtcaccacatatggagtcatcatgaagcttgtgcctgctgtcctggccagtccaaagtccaggattttcaatgtgcaatcagacttgactacaatgttacttggttttaaatccctgtgaataattccagcagaatggaggtgcttaatgccacacaacatttggtacagcaggtaagacattcgctcatggtctaattccatctgaatcacttgacataagttggcatccatcagttccattactaagtaaacatcttggaactcctccagcgttttctggggtgtgaagacatttaataaactaataatgtttttatggttcacacacttcatgaggaccagctcccggtacgctctcttggcatgtgtttggttctgaaagggtctgctgagcttcttaatggccacatttctgtcaaggacagcatcatacgcggcacaaactatgccctgagccccagagccaataggctttagattctggtagcgcttgagaactgtgaaggttgagtctcccacttccacactgtagaactggttgtcaactttgcttttgctcatgttgtaatgtttggcaatatatgacacatccacttgtttatcgaatcccttgttttacctgtaaggaacacacacctgacaaaaggcaattttcacatccaatgttggttcactgcagtagtataagaaatggaggctcataaataccacagcttgtatggtttctcatctataggaaacgggtctaattcaacagtttcttgcataagttgccatagtgaagatctgagatgggcctgctgttggtgtttctcacactagccagaggcagccaaaccgctacatccaaagcatccagcccctaaaatctaa

SEQ ID NO: 9191 - RNA, 4455 nt, Homo sapiens
  source 1..4455: mol_type = other RNA
agacagtagttcttgcctggtttactctgagggggaaattcaccacttatgcaggtacgagagatagcctgtcaagcactttgaagatgctggctggagacttccttctgtcttgtgatgtcatcttgcggctgatgaaattccccttgagactctctttaaagcagcttcctgctctccgcacttaatcccatgtggtataaagtaagggaggggagaagccacagatatatcaagagaaaagtaccgagaaagaaaatcagtaaagaattagagatacagagaggagaagtttttaaaaaaaaaaaaaaaaaacaggaatatgaaagagagggagctcaagtgactgaggaggcatttttaacaatcaggttatctgcaatattaaccagaaaaaaaatggtagcaaaatagagaaaatgggccatttttattccaggggacaagctgcacaaaggaatgttcttctatttattttaaacaaatgactgcgtgtactgaatctgactgtgtgaaataatctcagaatggcagcaccactggcatggcgatggtgcaggtgggtgcagttccctgtggtctctattgcttgaagagagaaagaaagttccctattattatatttaaggcagttttcagagcactggcattcttgtttgctctgttttggggatattctatttgccaatcagttcacactcatcaaccatccacttcctgtctttcacttcttcaggtgaaatatcaccactctagtgagcaccaacatggtcagagtgcaaataactgtgatggatacttcgaagtgaataagaagggaagcctgattattgctgagatcaccttggtattgccttgtacataaccaagatgtttcacagtgcctccttaagtgctcaggaaagcactttcatttaatttaatttaagctaaattctggagattttgctaaacattgacattaatgcttcatggcttttaagacaaactcatattgctaaaactatttggcagcagtaaatttatgggcagagttattgctcttacatctactgcagtacaaaactcagatgatcagcccttcgattgctcatacttattaaaataaataaataaacatgaaacatcagccacattaaggagtcagggaaactcctgaggaataacaatgtctctggagatgttttcaaatgctaacctgagactcacactgtggtttgggggtttcattattattattattattttatttcagaagaggaaagtaatattatttctcaaaataaaactttggcagagtatgaatcagggaagcagcccacacatggaaaacacaatccacaatctgaaagtagtctaggcaggctcatttttttgttgaaggaattcacatggaggcaattctgctcagttccagagagagattcttatcatcaaaagcacacacaataaccttgcttcaccacctgccactttctccagtggcctcttgttgtgaccagtaattgagaaatgacaaatgggtatagagccaaatctctaaaacagggacaccagtgtctcctagtatctgggtaataacctcctttcagtcttagtccacaccacacactaccctccagtctctcctactctttactgtcacagaaaagactctcagcttttattcacacctgccttcagaaggccaaaccattttgtgcctgaaaactgttacccactcgccccacactttacataagtatcacatatgttctttctacaaattggtatacaggtgccatttaatccattcaaatttggaagctacatcttcaagggtctgagagagctcactccccccatatattccccctttacatgttttcttataagacatacagtttaatcaattaacaaactaaacagcttatatactggcaatatattacagatgggtttatgtcagagtaatagatcacatgaaatggaccatgtggtaccccagtgcattatgtcttggtagagccctgaggacactgacagtagcatctctaagtaagtagtgctgtatgaatacagacacatgcggatctgtatctacatccatctgactaggccaaggagcaggtagatgcaagatagagacacacacatgctggatggggccactgcacaccttgtcatgccatttaaaagggcagttacaggttgccggttttgcagccattaaaattacactttatggaaaaggcttctctaattgtgtctgatttgctttctgtagtaagcatcattggaagaagaccaaagcaagagcaactagaagttaaatatacatttgagcttagctgcaatacagaaccctggggaagaagcaggctgaaagatttatttaattttaggcttggattctctcccttgctgttttcttgatgttgtgtgtctgcatttgtgtgtgtgtgtgtgtctgcgtgtgtgtgtgttccatcacatcatctcctgaagaacgctgggtttcgcaggcaggcggctagtcacctgcaacaacccaggggtcctgccgaggcttccaggctgctgtcagtgtcagatgccagggtctggtcggtggacatggaggagatgtcattgacagacgaggatggagggagactctcactgctgttcactgctgcacctgaaggagaaggctgtccttttactacaccatttttagtcttttcttctgaattcattacttccttgtagataagttctttccattcttcaattgtgtgttctctttcatccaactgcttgtcatatatctgaggtggaggcgcctccacttcggctgggtcataccagacgttgatgtagggatgctgtaaggcgtcgtccactgatattctttttgctgggtcaatcactagcatctttgacaacaagtccctggcttggctggctttgagtttattgtgctcggagtccgctgggaagagggaatctgggaagagtttggggaaggtgagtcccgcatacttgggccgattctccacatagtttcttactgtgggttgcaatttcttcatgaattctggacatggtgttcctagttgttcaattaccttattccactggtcaatatagtcccttcctggaaagaggattttgtggcgaaccatttctcccataatgcatcccacagaccatatatccacgttctccttgtagcccatccccaggatgacctcaggggctctgtaataacgtgtcaccacatatggagtcatcatgaagcttgtgcctgctgtcctggccagtccaaagtccaggattttcaatgtgcaatcagacttgactacaatgttacttggttttaaatccctgtgaataattccagcagaatggaggtgcttaatgccacacaacatttggtacagcaggtaagacattcgctcatggtctaattccatctgaatcacttgacataagttggcatccatcagttccattactaagtaaacatcttggaactcctccagcgttttctggggtgtgaagacatttaataaactaataatgtttttatggttcacacacttcatgaggaccagctcccggtacgctctcttggcatgtgtttggttctgaaagggtctgctgagcttcttaatggccacatttctgtcaaggacagcatcatacgcggcacaaactatgccctgagccccagagccaataggctttagattctggtagcgcttgagaactgtgaaggttgagtctcccacttccacactgtagaactggttgtcaactttgcttttgctcatgttgtaatgtttggcaatatatgacacatccacttgtttatcgaatcccttgttttacctgtaaggaacacacacctgacaaaaggcaattttcacatccaatgttggttcactgcagtagtataagaaatggaggctcataaataccacagcttgtatggtttctcatctataggaaacgggtctaattcaacagtttcttgcataagttgccatagtgaagatctgagatgggcctgctgttggtgtttctcacactagccattccgtgcctgagaactacgatcctgatccggcagtgtttgccccagaaatcctccctacttgtttttcattaaccacattccagactaacatggaagagattctttggagatatggagattgtttaaaattaacgatggacaggtgatttccaagaaaacccaatcttaaactcactcaagcccctaggaattgaggggtgaggacaaaaaaggaaatttgtaaaaatgaaaaaagaaaagaaaaaggtaagcatatagcaagcaccacccacccccataaaaataaaaagtgaaggggaggttaaagaaaatagaagaagagtggcttgctgaatcaccctctttcactgcctggaaaccattgtgcagcgtgatgctgcctgtaccattgt

SEQ ID NO: 9192 - RNA, 4364 nt, Homo sapiens
  source 1..4364: mol_type = other RNA
agacagtagttcttgcctggtttactctgagggggaaattcaccacttatgcaggtacgagagatagcctgtcaagcactttgaagatgctggctggagacttccttctgtcttgtgatgtcatcttgcggctgatgaaattccccttgagactctctttaaagcagcttcctgctctccgcacttaatcccatgtggtataaagtaagggaggggagaagccacagatatatcaagagaaaagtaccgagaaagaaaatcagtaaagaattagagatacagagaggagaagtttttaaaaaaaaaaaaaaaaaacaggaatatgaaagagagggagctcaagtgactgaggaggcatttttaacaatcaggttatctgcaatattaaccagaaaaaaaatggtagcaaaatagagaaaatgggccatttttattccaggggacaagctgcacaaaggaatgttcttctatttattttaaacaaatgactgcgtgtactgaatctgactgtgtgaaataatctcagaatggcagcaccactggcatggcgatggtgcaggtgggtgcagttccctgtggtctctattgcttgaagagagaaagaaagttccctattattatatttaaggcagttttcagagcactggcattcttgtttgctctgttttggggatattctatttgccaatcagttcacactcatcaaccatccacttcctgtctttcacttcttcaggtgaaatatcaccactctagtgagcaccaacatggtcagagtgcaaataactgtgatggatacttcgaagtgaataagaagggaagcctgattattgctgagatcaccttggtattgccttgtacataaccaagatgtttcacagtgcctccttaagtgctcaggaaagcactttcatttaatttaatttaagctaaattctggagattttgctaaacattgacattaatgcttcatggcttttaagacaaactcatattgctaaaactatttggcagcagtaaatttatgggcagagttattgctcttacatctactgcagtacaaaactcagatgatcagcccttcgattgctcatacttattaaaataaataaataaacatgaaacatcagccacattaaggagtcagggaaactcctgaggaataacaatgtctctggagatgttttcaaatgctaacctgagactcacactgtggtttgggggtttcattattattattattattttatttcagaagaggaaagtaatattatttctcaaaataaaactttggcagagtatgaatcagggaagcagcccacacatggaaaacacaatccacaatctgaaagtagtctaggcaggctcatttttttgttgaaggaattcacatggaggcaattctgctcagttccagagagagattcttatcatcaaaagcacacacaataaccttgcttcaccacctgccactttctccagtggcctcttgttgtgaccagtaattgagaaatgacaaatgggtatagagccaaatctctaaaacagggacaccagtgtctcctagtatctgggtaataacctcctttcagtcttagtccacaccacacactaccctccagtctctcctactctttactgtcacagaaaagactctcagcttttattcacacctgccttcagaaggccaaaccattttgtgcctgaaaactgttacccactcgccccacactttacataagtatcacatatgttctttctacaaattggtatacaggtgccatttaatccattcaaatttggaagctacatcttcaagggtctgagagagctcactccccccatatattccccctttacatgttttcttataagacatacagtttaatcaattaacaaactaaacagcttatatactggcaatatattacagatgggtttatgtcagagtaatagatcacatgaaatggaccatgtggtaccccagtgcattatgtcttggtagagccctgaggacactgacagtagcatctctaagtaagtagtgctgtatgaatacagacacatgcggatctgtatctacatccatctgactaggccaaggagcaggtagatgcaagatagagacacacacatgctggatggggccactgcacaccttgtcatgccatttaaaagggcagttacaggttgccggttttgcagccattaaaattacactttatggaaaaggcttctctaattgtgtctgatttgctttctgtagtaagcatcattggaagaagaccaaagcaagagcaactagaagttaaatatacatttgagcttagctgcaatacagaaccctggggaagaagcaggctgaaagatttatttaattttaggcttggattctctcccttgctgttttcttgatgttgtgtgtctgcatttgtgtgtgtgtgtgtgtctgcgtgtgtgtgtgttccatcacatcatctcctgaagaacgctgggtttcgcaggcaggcggctagtcacctgcaacaacccaggggtcctgccgaggcttccaggctgctgtcagtgtcagatgccagggtctggtcggtggacatggaggagatgtcattgacagacgaggatggagggagactctcactgctgttcactgctgcacctgaaggagaaggctgtccttttactacaccatttttagtcttttcttctgaattcattacttccttgtagataagttctttccattcttcaattgtgtgttctctttcatccaactgcttgtcatatatctgaggtggaggcgcctccacttcggctgggtcataccagacgttgatgtagggatgctgtaaggcgtcgtccactgatattctttttgctgggtcaatcactagcatctttgacaacaagtccctggcttggctggctttgagtttattgtgctcggagtccgctgggaagagggaatctgggaagagtttggggaaggtgagtcccgcatacttgggccgattctccacatagtttcttactgtgggttgcaatttcttcatgaattctggacatggtgttcctagttgttcaattaccttattccactggtcaatatagtcccttcctggaaagaggattttgtggcgaaccatttctcccataatgcatcccacagaccatatatccacgttctccttgtagcccatccccaggatgacctcaggggctctgtaataacgtgtcaccacatatggagtcatcatgaagcttgtgcctgctgtcctggccagtccaaagtccaggattttcaatgtgcaatcagacttgactacaatgttacttggttttaaatccctgtgaataattccagcagaatggaggtgcttaatgccacacaacatttggtacagcaggtaagacattcgctcatggtctaattccatctgaatcacttgacataagttggcatccatcagttccattactaagtaaacatcttggaactcctccagcgttttctggggtgtgaagacatttaataaactaataatgtttttatggttcacacacttcatgaggaccagctcccggtacgctctcttggcatgtgtttggttctgaaagggtctgctgagcttcttaatggccacatttctgtcaaggacagcatcatacgcggcacaaactatgccctgagccccagagccaataggctttagattctggtagcgcttgagaactgtgaaggttgagtctcccacttccacactgtagaactggttgtcaactttgcttttgctcatgttgtaatgtttggcaatatatgacacatccacttgtttatcgaatcccttgttttacctgtaaggaacacacacctgacaaaaggcaattttcacatccaatgttggttcactgcagtagtataagaaatggaggctcataaataccacagcttgtatggtttctcatctataggaaacgggtctaattcaacagtttcttgcataagttgccatagtgaagatctgagatgggcctgctgttggtgtttctcacactagcctaaagtagaaaattcacagaagcttctctgagagaaatggtccttactgcaactattttaaatatgttgataagcattctgtgttatcttccagggtccgacaactagccgatgagggatagaaggagatattggatgttgtgctggcaatgcctggtgcacttacactcgttttccttccacctgaactgtagtctatcccatatgacttagcctgcttccttgcagtttgttcataaaagttatcatcaacatggccagaagcaggcagggctgctgtacagacactgtcaggctctgcacc

SEQ ID NO: 9193 - RNA, 4260 nt, Homo sapiens
  source 1..4260: mol_type = other RNA
agacagtagttcttgcctggtttactctgagggggaaattcaccacttatgcaggtacgagagatagcctgtcaagcactttgaagatgctggctggagacttccttctgtcttgtgatgtcatcttgcggctgatgaaattccccttgagactctctttaaagcagcttcctgctctccgcacttaatcccatgtggtataaagtaagggaggggagaagccacagatatatcaagagaaaagtaccgagaaagaaaatcagtaaagaattagagatacagagaggagaagtttttaaaaaaaaaaaaaaaaaacaggaatatgaaagagagggagctcaagtgactgaggaggcatttttaacaatcaggttatctgcaatattaaccagaaaaaaaatggtagcaaaatagagaaaatgggccatttttattccaggggacaagctgcacaaaggaatgttcttctatttattttaaacaaatgactgcgtgtactgaatctgactgtgtgaaataatctcagaatggcagcaccactggcatggcgatggtgcaggtgggtgcagttccctgtggtctctattgcttgaagagagaaagaaagttccctattattatatttaaggcagttttcagagcactggcattcttgtttgctctgttttggggatattctatttgccaatcagttcacactcatcaaccatccacttcctgtctttcacttcttcaggtgaaatatcaccactctagtgagcaccaacatggtcagagtgcaaataactgtgatggatacttcgaagtgaataagaagggaagcctgattattgctgagatcaccttggtattgccttgtacataaccaagatgtttcacagtgcctccttaagtgctcaggaaagcactttcatttaatttaatttaagctaaattctggagattttgctaaacattgacattaatgcttcatggcttttaagacaaactcatattgctaaaactatttggcagcagtaaatttatgggcagagttattgctcttacatctactgcagtacaaaactcagatgatcagcccttcgattgctcatacttattaaaataaataaataaacatgaaacatcagccacattaaggagtcagggaaactcctgaggaataacaatgtctctggagatgttttcaaatgctaacctgagactcacactgtggtttgggggtttcattattattattattattttatttcagaagaggaaagtaatattatttctcaaaataaaactttggcagagtatgaatcagggaagcagcccacacatggaaaacacaatccacaatctgaaagtagtctaggcaggctcatttttttgttgaaggaattcacatggaggcaattctgctcagttccagagagagattcttatcatcaaaagcacacacaataaccttgcttcaccacctgccactttctccagtggcctcttgttgtgaccagtaattgagaaatgacaaatgggtatagagccaaatctctaaaacagggacaccagtgtctcctagtatctgggtaataacctcctttcagtcttagtccacaccacacactaccctccagtctctcctactctttactgtcacagaaaagactctcagcttttattcacacctgccttcagaaggccaaaccattttgtgcctgaaaactgttacccactcgccccacactttacataagtatcacatatgttctttctacaaattggtatacaggtgccatttaatccattcaaatttggaagctacatcttcaagggtctgagagagctcactccccccatatattccccctttacatgttttcttataagacatacagtttaatcaattaacaaactaaacagcttatatactggcaatatattacagatgggtttatgtcagagtaatagatcacatgaaatggaccatgtggtaccccagtgcattatgtcttggtagagccctgaggacactgacagtagcatctctaagtaagtagtgctgtatgaatacagacacatgcggatctgtatctacatccatctgactaggccaaggagcaggtagatgcaagatagagacacacacatgctggatggggccactgcacaccttgtcatgccatttaaaagggcagttacaggttgccggttttgcagccattaaaattacactttatggaaaaggcttctctaattgtgtctgatttgctttctgtagtaagcatcattggaagaagaccaaagcaagagcaactagaagttaaatatacatttgagcttagctgcaatacagaaccctggggaagaagcaggctgaaagatttatttaattttaggcttggattctctcccttgctgttttcttgatgttgtgtgtctgcatttgtgtgtgtgtgtgtgtctgcgtgtgtgtgtgttccatcacatcatctcctgaagaacgctgggtttcgcaggcaggcggctagtcacctgcaacaacccaggggtcctgccgaggcttccaggctgctgtcagtgtcagatgccagggtctggtcggtggacatggaggagatgtcattgacagacgaggatggagggagactctcactgctgttcactgctgcacctgaaggagaaggctgtccttttactacaccatttttagtcttttcttctgaattcattacttccttgtagataagttctttccattcttcaattgtgtgttctctttcatccaactgcttgtcatatatctgaggtggaggcgcctccacttcggctgggtcataccagacgttgatgtagggatgctgtaaggcgtcgtccactgatattctttttgctgggtcaatcactagcatctttgacaacaagtccctggcttggctggctttgagtttattgtgctcggagtccgctgggaagagggaatctgggaagagtttggggaaggtgagtcccgcatacttgggccgattctccacatagtttcttactgtgggttgcaatttcttcatgaattctggacatggtgttcctagttgttcaattaccttattccactggtcaatatagtcccttcctggaaagaggattttgtggcgaaccatttctcccataatgcatcccacagaccatatatccacgttctccttgtagcccatccccaggatgacctcaggggctctgtaataacgtgtcaccacatatggagtcatcatgaagcttgtgcctgctgtcctggccagtccaaagtccaggattttcaatgtgcaatcagacttgactacaatgttacttggttttaaatccctgtgaataattccagcagaatggaggtgcttaatgccacacaacatttggtacagcaggtaagacattcgctcatggtctaattccatctgaatcacttgacataagttggcatccatcagttccattactaagtaaacatcttggaactcctccagcgttttctggggtgtgaagacatttaataaactaataatgtttttatggttcacacacttcatgaggaccagctcccggtacgctctcttggcatgtgtttggttctgaaagggtctgctgagcttcttaatggccacatttctgtcaaggacagcatcatacgcggcacaaactatgccctgagccccagagccaataggctttagattctggtagcgcttgagaactgtgaaggttgagtctcccacttccacactgtagaactggttgtcaactttgcttttgctcatgttgtaatgtttggcaatatatgacacatccacttgtttatcgaatcccttgttttacctgtaaggaacacacacctgacaaaaggcaattttcacatccaatgttggttcactgcagtagtataagaaatggaggctcataaataccacagcttgtatggtttctcatctataggaaacgggtctaattcaacagtttcttgcataagttgccatagtgaagatctgagatgggcctgctgttggtgtttctcacactagcgcatttttcactctcctcctcactccctagggtcatagttttgattctgaagttagaagtgtgggggtcgtcggctgcattttcaacttggcctaaaagttggagttcaccacactgcaggcgctaggaactctgccgctcggtcaccaacctgagcctctggctagtccgaagaacgcgaaaagccaggcccaaggcact

SEQ ID NO: 9194 - RNA, 4258 nt, Homo sapiens
  source 1..4258: mol_type = other RNA
agacagtagttcttgcctggtttactctgagggggaaattcaccacttatgcaggtacgagagatagcctgtcaagcactttgaagatgctggctggagacttccttctgtcttgtgatgtcatcttgcggctgatgaaattccccttgagactctctttaaagcagcttcctgctctccgcacttaatcccatgtggtataaagtaagggaggggagaagccacagatatatcaagagaaaagtaccgagaaagaaaatcagtaaagaattagagatacagagaggagaagtttttaaaaaaaaaaaaaaaaaacaggaatatgaaagagagggagctcaagtgactgaggaggcatttttaacaatcaggttatctgcaatattaaccagaaaaaaaatggtagcaaaatagagaaaatgggccatttttattccaggggacaagctgcacaaaggaatgttcttctatttattttaaacaaatgactgcgtgtactgaatctgactgtgtgaaataatctcagaatggcagcaccactggcatggcgatggtgcaggtgggtgcagttccctgtggtctctattgcttgaagagagaaagaaagttccctattattatatttaaggcagttttcagagcactggcattcttgtttgctctgttttggggatattctatttgccaatcagttcacactcatcaaccatccacttcctgtctttcacttcttcaggtgaaatatcaccactctagtgagcaccaacatggtcagagtgcaaataactgtgatggatacttcgaagtgaataagaagggaagcctgattattgctgagatcaccttggtattgccttgtacataaccaagatgtttcacagtgcctccttaagtgctcaggaaagcactttcatttaatttaatttaagctaaattctggagattttgctaaacattgacattaatgcttcatggcttttaagacaaactcatattgctaaaactatttggcagcagtaaatttatgggcagagttattgctcttacatctactgcagtacaaaactcagatgatcagcccttcgattgctcatacttattaaaataaataaataaacatgaaacatcagccacattaaggagtcagggaaactcctgaggaataacaatgtctctggagatgttttcaaatgctaacctgagactcacactgtggtttgggggtttcattattattattattattttatttcagaagaggaaagtaatattatttctcaaaataaaactttggcagagtatgaatcagggaagcagcccacacatggaaaacacaatccacaatctgaaagtagtctaggcaggctcatttttttgttgaaggaattcacatggaggcaattctgctcagttccagagagagattcttatcatcaaaagcacacacaataaccttgcttcaccacctgccactttctccagtggcctcttgttgtgaccagtaattgagaaatgacaaatgggtatagagccaaatctctaaaacagggacaccagtgtctcctagtatctgggtaataacctcctttcagtcttagtccacaccacacactaccctccagtctctcctactctttactgtcacagaaaagactctcagcttttattcacacctgccttcagaaggccaaaccattttgtgcctgaaaactgttacccactcgccccacactttacataagtatcacatatgttctttctacaaattggtatacaggtgccatttaatccattcaaatttggaagctacatcttcaagggtctgagagagctcactccccccatatattccccctttacatgttttcttataagacatacagtttaatcaattaacaaactaaacagcttatatactggcaatatattacagatgggtttatgtcagagtaatagatcacatgaaatggaccatgtggtaccccagtgcattatgtcttggtagagccctgaggacactgacagtagcatctctaagtaagtagtgctgtatgaatacagacacatgcggatctgtatctacatccatctgactaggccaaggagcaggtagatgcaagatagagacacacacatgctggatggggccactgcacaccttgtcatgccatttaaaagggcagttacaggttgccggttttgcagccattaaaattacactttatggaaaaggcttctctaattgtgtctgatttgctttctgtagtaagcatcattggaagaagaccaaagcaagagcaactagaagttaaatatacatttgagcttagctgcaatacagaaccctggggaagaagcaggctgaaagatttatttaattttaggcttggattctctcccttgctgttttcttgatgttgtgtgtctgcatttgtgtgtgtgtgtgtgtctgcgtgtgtgtgtgttccatcacatcatctcctgaagaacgctgggtttcgcaggcaggcggctagtcacctgcaacaacccaggggtcctgccgaggcttccaggctgctgtcagtgtcagatgccagggtctggtcggtggacatggaggagatgtcattgacagacgaggatggagggagactctcactgctgttcactgctgcacctgaaggagaaggctgtccttttactacaccatttttagtcttttcttctgaattcattacttccttgtagataagttctttccattcttcaattgtgtgttctctttcatccaactgcttgtcatatatctgaggtggaggcgcctccacttcggctgggtcataccagacgttgatgtagggatgctgtaaggcgtcgtccactgatattctttttgctgggtcaatcactagcatctttgacaacaagtccctggcttggctggctttgagtttattgtgctcggagtccgctgggaagagggaatctgggaagagtttggggaaggtgagtcccgcatacttgggccgattctccacatagtttcttactgtgggttgcaatttcttcatgaattctggacatggtgttcctagttgttcaattaccttattccactggtcaatatagtcccttcctggaaagaggattttgtggcgaaccatttctcccataatgcatcccacagaccatatatccacgttctccttgtagcccatccccaggatgacctcaggggctctgtaataacgtgtcaccacatatggagtcatcatgaagcttgtgcctgctgtcctggccagtccaaagtccaggattttcaatgtgcaatcagacttgactacaatgttacttggttttaaatccctgtgaataattccagcagaatggaggtgcttaatgccacacaacatttggtacagcaggtaagacattcgctcatggtctaattccatctgaatcacttgacataagttggcatccatcagttccattactaagtaaacatcttggaactcctccagcgttttctggggtgtgaagacatttaataaactaataatgtttttatggttcacacacttcatgaggaccagctcccggtacgctctcttggcatgtgtttggttctgaaagggtctgctgagcttcttaatggccacatttctgtcaaggacagcatcatacgcggcactgacaaaaggcaattttcacatccaatgttggttcactgcagtagtataagaaatggaggctcataaataccacagcttgtatggtttctcatctataggaaacgggtctaattcaacagtttcttgcataagttgccatagtgaagatctgagatgggcctgctgttggtgtttctcacactagccattccgtgcctgagaactacgatcctgatccggcagtgtttgccccagaaatcctccctacttgtttttcattaaccacattccagactaacatggaagagattctttggagatatggagattgtttaaaattaacgatggacaggtgatttccaagaaaacccaatcttaaactcactcaagcccctaggaattgaggggtgaggacaaaaaaggaaatttgtaaaaatgaaaaaagaaaagaaaaaggtaagcatatagcaagcaccacccacccccataaaaataaaaagtgaaggggaggttaaagaaaatagaagaagagtggcttgctgaatcaccctctttcactgcctggaaaccattgtgcagcgtgatgctgcctgtaccattgt

SEQ ID NO: 9195 - RNA, 4419 nt, Homo sapiens
  source 1..4419: mol_type = other RNA
agacagtagttcttgcctggtttactctgagggggaaattcaccacttatgcaggtacgagagatagcctgtcaagcactttgaagatgctggctggagacttccttctgtcttgtgatgtcatcttgcggctgatgaaattccccttgagactctctttaaagcagcttcctgctctccgcacttaatcccatgtggtataaagtaagggaggggagaagccacagatatatcaagagaaaagtaccgagaaagaaaatcagtaaagaattagagatacagagaggagaagtttttaaaaaaaaaaaaaaaaaacaggaatatgaaagagagggagctcaagtgactgaggaggcatttttaacaatcaggttatctgcaatattaaccagaaaaaaaatggtagcaaaatagagaaaatgggccatttttattccaggggacaagctgcacaaaggaatgttcttctatttattttaaacaaatgactgcgtgtactgaatctgactgtgtgaaataatctcagaatggcagcaccactggcatggcgatggtgcaggtgggtgcagttccctgtggtctctattgcttgaagagagaaagaaagttccctattattatatttaaggcagttttcagagcactggcattcttgtttgctctgttttggggatattctatttgccaatcagttcacactcatcaaccatccacttcctgtctttcacttcttcaggtgaaatatcaccactctagtgagcaccaacatggtcagagtgcaaataactgtgatggatacttcgaagtgaataagaagggaagcctgattattgctgagatcaccttggtattgccttgtacataaccaagatgtttcacagtgcctccttaagtgctcaggaaagcactttcatttaatttaatttaagctaaattctggagattttgctaaacattgacattaatgcttcatggcttttaagacaaactcatattgctaaaactatttggcagcagtaaatttatgggcagagttattgctcttacatctactgcagtacaaaactcagatgatcagcccttcgattgctcatacttattaaaataaataaataaacatgaaacatcagccacattaaggagtcagggaaactcctgaggaataacaatgtctctggagatgttttcaaatgctaacctgagactcacactgtggtttgggggtttcattattattattattattttatttcagaagaggaaagtaatattatttctcaaaataaaactttggcagagtatgaatcagggaagcagcccacacatggaaaacacaatccacaatctgaaagtagtctaggcaggctcatttttttgttgaaggaattcacatggaggcaattctgctcagttccagagagagattcttatcatcaaaagcacacacaataaccttgcttcaccacctgccactttctccagtggcctcttgttgtgaccagtaattgagaaatgacaaatgggtatagagccaaatctctaaaacagggacaccagtgtctcctagtatctgggtaataacctcctttcagtcttagtccacaccacacactaccctccagtctctcctactctttactgtcacagaaaagactctcagcttttattcacacctgccttcagaaggccaaaccattttgtgcctgaaaactgttacccactcgccccacactttacataagtatcacatatgttctttctacaaattggtatacaggtgccatttaatccattcaaatttggaagctacatcttcaagggtctgagagagctcactccccccatatattccccctttacatgttttcttataagacatacagtttaatcaattaacaaactaaacagcttatatactggcaatatattacagatgggtttatgtcagagtaatagatcacatgaaatggaccatgtggtaccccagtgcattatgtcttggtagagccctgaggacactgacagtagcatctctaagtaagtagtgctgtatgaatacagacacatgcggatctgtatctacatccatctgactaggccaaggagcaggtagatgcaagatagagacacacacatgctggatggggccactgcacaccttgtcatgccatttaaaagggcagttacaggttgccggttttgcagccattaaaattacactttatggaaaaggcttctctaattgtgtctgatttgctttctgtagtaagcatcattggaagaagaccaaagcaagagcaactagaagttaaatatacatttgagcttagctgcaatacagaaccctggggaagaagcaggctgaaagatttatttaattttaggcttggattctctcccttgctgttttcttgatgttgtgtgtctgcatttgtgtgtgtgtgtgtgtctgcgtgtgtgtgtgttccatcacatcatctcctgaagaacgctgggtttcgcaggcaggcggctagtcacctgcaacaacccaggggtcctgccgaggcttccaggctgctgtcagtgtcagatgccagggtctggtcggtggacatggaggagatgtcattgacagacgaggatggagggagactctcactgctgttcactgctgcacctgaaggagaaggctgtccttttactacaccatttttagtcttttcttctgaattcattacttccttgtagataagttctttccattcttcaattgtgtgttctctttcatccaactgcttgtcatatatctgaggtggaggcgcctccacttcggctgggtcataccagacgttgatgtagggatgctgtaaggcgtcgtccactgatattctttttgctgggtcaatcactagcatctttgacaacaagtccctggcttggctggctttgagtttattgtgctcggagtccgctgggaagagggaatctgggaagagtttggggaaggtgagtcccgcatacttgggccgattctccacatagtttcttactgtgggttgcaatttcttcatgaattctggacatggtgttcctagttgttcaattaccttattccactggtcaatatagtcccttcctggaaagaggattttgtggcgaaccatttctcccataatgcatcccacagaccatatatccacgttctccttgtagcccatccccaggatgacctcaggggctctgtaataacgtgtcaccacatatggagtcatcatgaagcttgtgcctgctgtcctggccagtccaaagtccaggattttcaatgtgcaatcagacttgactacaatgttacttggttttaaatccctgtgaataattccagcagaatggaggtgcttaatgccacacaacatttggtacagcaggtaagacattcgctcatggtctaattccatctgaatcacttgacataagttggcatccatcagttccattactaagtaagtttttatggttcacacacttcatgaggaccagctcccggtacgctctcttggcatgtgtttggttctgaaagggtctgctgagcttcttaatggccacatttctgtcaaggacagcatcatacgcggcacaaactatgccctgagccccagagccaataggctttagattctggtagcgcttgagaactgtgaaggttgagtctcccacttccacactgtagaactggttgtcaactttgcttttgctcatgttgtaatgtttggcaatatatgacacatccacttgtttatcgaatccctgacaaaaggcaattttcacatccaatgttggttcactgcagtagtataagaaatggaggctcataaataccacagcttgtatggtttctcatctataggaaacgggtctaattcaacagtttcttgcataagttgccatagtgaagatctgagatgggcctgctgttggtgtttctcacactagccattccgtgcctgagaactacgatcctgatccggcagtgtttgccccagaaatcctccctacttgtttttcattaaccacattccagactaacatggaagagattctttggagatatggagattgtttaaaattaacgatggacaggtgatttccaagaaaacccaatcttaaactcactcaagcccctaggaattgaggggtgaggacaaaaaaggaaatttgtaaaaatgaaaaaagaaaagaaaaaggtaagcatatagcaagcaccacccacccccataaaaataaaaagtgaaggggaggttaaagaaaatagaagaagagtggcttgctgaatcaccctctttcactgcctggaaaccattgtgcagcgtgatgctgcctgtaccattgtggaacctaccagaggagacggacagagggcttggggaatggggttgctat

SEQ ID NO: 9196 - RNA, 4396 nt, Homo sapiens
  source 1..4396: mol_type = other RNA
agacagtagttcttgcctggtttactctgagggggaaattcaccacttatgcaggtacgagagatagcctgtcaagcactttgaagatgctggctggagacttccttctgtcttgtgatgtcatcttgcggctgatgaaattccccttgagactctctttaaagcagcttcctgctctccgcacttaatcccatgtggtataaagtaagggaggggagaagccacagatatatcaagagaaaagtaccgagaaagaaaatcagtaaagaattagagatacagagaggagaagtttttaaaaaaaaaaaaaaaaaacaggaatatgaaagagagggagctcaagtgactgaggaggcatttttaacaatcaggttatctgcaatattaaccagaaaaaaaatggtagcaaaatagagaaaatgggccatttttattccaggggacaagctgcacaaaggaatgttcttctatttattttaaacaaatgactgcgtgtactgaatctgactgtgtgaaataatctcagaatggcagcaccactggcatggcgatggtgcaggtgggtgcagttccctgtggtctctattgcttgaagagagaaagaaagttccctattattatatttaaggcagttttcagagcactggcattcttgtttgctctgttttggggatattctatttgccaatcagttcacactcatcaaccatccacttcctgtctttcacttcttcaggtgaaatatcaccactctagtgagcaccaacatggtcagagtgcaaataactgtgatggatacttcgaagtgaataagaagggaagcctgattattgctgagatcaccttggtattgccttgtacataaccaagatgtttcacagtgcctccttaagtgctcaggaaagcactttcatttaatttaatttaagctaaattctggagattttgctaaacattgacattaatgcttcatggcttttaagacaaactcatattgctaaaactatttggcagcagtaaatttatgggcagagttattgctcttacatctactgcagtacaaaactcagatgatcagcccttcgattgctcatacttattaaaataaataaataaacatgaaacatcagccacattaaggagtcagggaaactcctgaggaataacaatgtctctggagatgttttcaaatgctaacctgagactcacactgtggtttgggggtttcattattattattattattttatttcagaagaggaaagtaatattatttctcaaaataaaactttggcagagtatgaatcagggaagcagcccacacatggaaaacacaatccacaatctgaaagtagtctaggcaggctcatttttttgttgaaggaattcacatggaggcaattctgctcagttccagagagagattcttatcatcaaaagcacacacaataaccttgcttcaccacctgccactttctccagtggcctcttgttgtgaccagtaattgagaaatgacaaatgggtatagagccaaatctctaaaacagggacaccagtgtctcctagtatctgggtaataacctcctttcagtcttagtccacaccacacactaccctccagtctctcctactctttactgtcacagaaaagactctcagcttttattcacacctgccttcagaaggccaaaccattttgtgcctgaaaactgttacccactcgccccacactttacataagtatcacatatgttctttctacaaattggtatacaggtgccatttaatccattcaaatttggaagctacatcttcaagggtctgagagagctcactccccccatatattccccctttacatgttttcttataagacatacagtttaatcaattaacaaactaaacagcttatatactggcaatatattacagatgggtttatgtcagagtaatagatcacatgaaatggaccatgtggtaccccagtgcattatgtcttggtagagccctgaggacactgacagtagcatctctaagtaagtagtgctgtatgaatacagacacatgcggatctgtatctacatccatctgactaggccaaggagcaggtagatgcaagatagagacacacacatgctggatggggccactgcacaccttgtcatgccatttaaaagggcagttacaggttgccggttttgcagccattaaaattacactttatggaaaaggcttctctaattgtgtctgatttgctttctgtagtaagcatcattggaagaagaccaaagcaagagcaactagaagttaaatatacatttgagcttagctgcaatacagaaccctggggaagaagcaggctgaaagatttatttaattttaggcttggattctctcccttgctgttttcttgatgttgtgtgtctgcatttgtgtgtgtgtgtgtgtctgcgtgtgtgtgtgttccatcacatcatctcctgaagaacgctgggtttcgcaggcaggcggctagtcacctgcaacaacccaggggtcctgccgaggcttccaggctgctgtcagtgtcagatgccagggtctggtcggtggacatggaggagatgtcattgacagacgaggatggagggagactctcactgctgttcactgctgcacctgaaggagaaggctgtccttttactacaccatttttagtcttttcttctgaattcattacttccttgtagataagttctttccattcttcaattgtgtgttctctttcatccaactgcttgtcatatatctgaggtggaggcgcctccacttcggctgggtcataccagacgttgatgtagggatgctgtaaggcgtcgtccactgatattctttttgctgggtcaatcactagcatctttgacaacaagtccctggcttggctggctttgagtttattgtgctcggagtccgctgggaagagggaatctgggaagagtttggggaaggtgagtcccgcatacttgggccgattctccacatagtttcttactgtgggttgcaatttcttcatgaattctggacatggtgttcctagttgttcaattaccttattccactggtcaatatagtcccttcctggaaagaggattttgtggcgaaccatttctcccataatgcatcccacagaccatatatccacgttctccttgtagcccatccccaggatgacctcaggggctctgtaataacgtgtcaccacatatggagtcatcatgaagcttgtgcctgctgtcctggccagtccaaagtccaggattttcaatgtgcaatcagacttgactacaatgttacttggttttaaatccctgtgaataattccagcagaatggaggtgcttaatgccacacaacatttggtacagcaggtaagacattcgctcatggtctaattccatctgaatcacttgacataagttggcatccatcagttccattactaagtaagtttttatggttcacacacttcatgaggaccagctcccggtacgctctcttggcatgtgtttggttctgaaagggtctgctgagcttcttaatggccacatttctgtcaaggacagcatcatacgcggcacaaactatgccctgagccccagagccaataggctttagattctggtagcgcttgagaactgtgaaggttgagtctcccacttccacactgtagaactggttgtcaactttgcttttgctcatgttgtaatgtttggcaatatatgacacatccacttgtttatcgaatcccttgttttacctgtaaggaacacacacctgacaaaaggcaattttcacatccaatgttggttcactgcagtagtataagaaatggaggctcataaataccacagcttgtatggtttctcatctataggaaacgggtctaattcaacagtttcttgcataagttgccatagtgaagatctgagatgggcctgctgttggtgtttctcacactagccattccgtgcctgagaactacgatcctgatccggcagtgtttgccccagaaatcctccctacttgtttttcattaaccacattccagactaacatggaagagattctttggagatatggagattgtttaaaattaacgatggacaggtgatttccaagaaaacccaatcttaaactcactcaagcccctaggaattgaggggtgaggacaaaaaaggaaatttgtaaaaatgaaaaaagaaaagaaaaaggtaagcatatagcaagcaccacccacccccataaaaataaaaagtgaaggggaggttaaagaaaatagaagaagagtggcttgctgaatcaccctctttcactgcctggaaaccattgtgcagcgtgatgctgcctgtaccattgt

SEQ ID NO: 9197 - RNA, 3845 nt, Homo sapiens
  source 1..3845: mol_type = other RNA
agacagtagttcttgcctggtttactctgagggggaaattcaccacttatgcaggtacgagagatagcctgtcaagcactttgaagatgctggctggagacttccttctgtcttgtgatgtcatcttgcggctgatgaaattccccttgagactctctttaaagcagcttcctgctctccgcacttaatcccatgtggtataaagtaagggaggggagaagccacagatatatcaagagaaaagtaccgagaaagaaaatcagtaaagaattagagatacagagaggagaagtttttaaaaaaaaaaaaaaaaaacaggaatatgaaagagagggagctcaagtgactgaggaggcatttttaacaatcaggttatctgcaatattaaccagaaaaaaaatggtagcaaaatagagaaaatgggccatttttattccaggggacaagctgcacaaaggaatgttcttctatttattttaaacaaatgactgcgtgtactgaatctgactgtgtgaaataatctcagaatggcagcaccactggcatggcgatggtgcaggtgggtgcagttccctgtggtctctattgcttgaagagagaaagaaagttccctattattatatttaaggcagttttcagagcactggcattcttgtttgctctgttttggggatattctatttgccaatcagttcacactcatcaaccatccacttcctgtctttcacttcttcaggtgaaatatcaccactctagtgagcaccaacatggtcagagtgcaaataactgtgatggatacttcgaagtgaataagaagggaagcctgattattgctgagatcaccttggtattgccttgtacataaccaagatgtttcacagtgcctccttaagtgctcaggaaagcactttcatttaatttaatttaagctaaattctggagattttgctaaacattgacattaatgcttcatggcttttaagacaaactcatattgctaaaactatttggcagcagtaaatttatgggcagagttattgctcttacatctactgcagtacaaaactcagatgatcagcccttcgattgctcatacttattaaaataaataaataaacatgaaacatcagccacattaaggagtcagggaaactcctgaggaataacaatgtctctggagatgttttcaaatgctaacctgagactcacactgtggtttgggggtttcattattattattattattttatttcagaagaggaaagtaatattatttctcaaaataaaactttggcagagtatgaatcagggaagcagcccacacatggaaaacacaatccacaatctgaaagtagtctaggcaggctcatttttttgttgaaggaattcacatggaggcaattctgctcagttccagagagagattcttatcatcaaaagcacacacaataaccttgcttcaccacctgccactttctccagtggcctcttgttgtgaccagtaattgagaaatgacaaatgggtatagagccaaatctctaaaacagggacaccagtgtctcctagtatctgggtaataacctcctttcagtcttagtccacaccacacactaccctccagtctctcctactctttactgtcacagaaaagactctcagcttttattcacacctgccttcagaaggccaaaccattttgtgcctgaaaactgttacccactcgccccacactttacataagtatcacatatgttctttctacaaattggtatacaggtgccatttaatccattcaaatttggaagctacatcttcaagggtctgagagagctcactccccccatatattccccctttacatgttttcttataagacatacagtttaatcaattaacaaactaaacagcttatatactggcaatatattacagatgggtttatgtcagagtaatagatcacatgaaatggaccatgtggtaccccagtgcattatgtcttggtagagccctgaggacactgacagtagcatctctaagtaagtagtgctgtatgaatacagacacatgcggatctgtatctacatccatctgactaggccaaggagcaggtagatgcaagatagagacacacacatgctggatggggccactgcacaccttgtcatgccatttaaaagggcagttacaggttgccggttttgcagccattaaaattacactttatggaaaaggcttctctaattgtgtctgatttgctttctgtagtaagcatcattggaagaagaccaaagcaagagcaactagaagttaaatatacatttgagcttagctgcaatacagaaccctggggaagaagcaggctgaaagatttatttaattttaggcttggattctctcccttgctgttttcttgatgttgtgtgtctgcatttgtgtgtgtgtgtgtgtctgcgtgtgtgtgtgttccatcacatcatctcctgaagaacgctgggtttcgcaggcaggcggctagtcacctgcaacaacccaggggtcctgccgaggcttccaggctgctgtcagtgtcagatgccagggtctggtcggtggacatggaggagatgtcattgacagacgaggatggagggagactctcactgctgttcactgctgcacctgaaggagaaggctgtccttttactacaccatttttagtcttttcttctgaattcattacttccttgtagataagttctttccattcttcaattgtgtgttctctttcatccaactgcttgtcatatatctgaggtggaggcgcctccacttcggctgggtcataccagacgttgatgtagggatgctgtaaggcgtcgtccactgatattctttttgctgggtcaatcactagcatctttgacaacaagtccctggcttggctggctttgagtttattgtgctcggagtccgctgggaagagggaatctgggaagagtttggggaaggtgagtcccgcatacttgggccgattctccacatagtttcttactgtgggttgcaatttcttcatgaattctggacatggtgttcctagttgttcaattaccttattccactggtcaatatcgttctccttgtagcccatccccaggatgacctcaggggctctgtaataacgtgtcaccacatatggagtcatcatgaagcttgtgcctgctgtcctggccagtccaaagtccaggattttcaatgtgcaatcagacttgactacaatgttacttggttttaaatccctgtgaataattccagcagaatggaggtgcttaatgccacacaacatttggtacagcaggtaagacattcgctcatggtctaattccatctgaatcacttgacataagttggcatccatcagttccattactaagtaaacatcttggaactcctccagcgttttctggggtgtgaagacatttaataaactaataatgtttttatggttcacacacttcatgaggaccagctcccggtacgctctcttggcatgtgtttggttctgaaagggtctgctgagcttcttaatggccacatttctgtcaaggacagcatcatacgcggcacaaactatgccctgagccccagagccaataggctttagattctggtagcgcttgagaactgtgaaggttgagtctcccacttccacactgtagaactggttgtcaactttgcttttgctcatgttgtaatgtttggcaatatatgacacatccacttgtttatcgaatccctgacaaaaggcaattttcacatccaatgttggttcactgcagtagtataagaaatggaggctcataaatac

SEQ ID NO: 9198 - RNA, 4384 nt, Homo sapiens
  source 1..4384: mol_type = other RNA
agacagtagttcttgcctggtttactctgagggggaaattcaccacttatgcaggtacgagagatagcctgtcaagcactttgaagatgctggctggagacttccttctgtcttgtgatgtcatcttgcggctgatgaaattccccttgagactctctttaaagcagcttcctgctctccgcacttaatcccatgtggtataaagtaagggaggggagaagccacagatatatcaagagaaaagtaccgagaaagaaaatcagtaaagaattagagatacagagaggagaagtttttaaaaaaaaaaaaaaaaaacaggaatatgaaagagagggagctcaagtgactgaggaggcatttttaacaatcaggttatctgcaatattaaccagaaaaaaaatggtagcaaaatagagaaaatgggccatttttattccaggggacaagctgcacaaaggaatgttcttctatttattttaaacaaatgactgcgtgtactgaatctgactgtgtgaaataatctcagaatggcagcaccactggcatggcgatggtgcaggtgggtgcagttccctgtggtctctattgcttgaagagagaaagaaagttccctattattatatttaaggcagttttcagagcactggcattcttgtttgctctgttttggggatattctatttgccaatcagttcacactcatcaaccatccacttcctgtctttcacttcttcaggtgaaatatcaccactctagtgagcaccaacatggtcagagtgcaaataactgtgatggatacttcgaagtgaataagaagggaagcctgattattgctgagatcaccttggtattgccttgtacataaccaagatgtttcacagtgcctccttaagtgctcaggaaagcactttcatttaatttaatttaagctaaattctggagattttgctaaacattgacattaatgcttcatggcttttaagacaaactcatattgctaaaactatttggcagcagtaaatttatgggcagagttattgctcttacatctactgcagtacaaaactcagatgatcagcccttcgattgctcatacttattaaaataaataaataaacatgaaacatcagccacattaaggagtcagggaaactcctgaggaataacaatgtctctggagatgttttcaaatgctaacctgagactcacactgtggtttgggggtttcattattattattattattttatttcagaagaggaaagtaatattatttctcaaaataaaactttggcagagtatgaatcagggaagcagcccacacatggaaaacacaatccacaatctgaaagtagtctaggcaggctcatttttttgttgaaggaattcacatggaggcaattctgctcagttccagagagagattcttatcatcaaaagcacacacaataaccttgcttcaccacctgccactttctccagtggcctcttgttgtgaccagtaattgagaaatgacaaatgggtatagagccaaatctctaaaacagggacaccagtgtctcctagtatctgggtaataacctcctttcagtcttagtccacaccacacactaccctccagtctctcctactctttactgtcacagaaaagactctcagcttttattcacacctgccttcagaaggccaaaccattttgtgcctgaaaactgttacccactcgccccacactttacataagtatcacatatgttctttctacaaattggtatacaggtgccatttaatccattcaaatttggaagctacatcttcaagggtctgagagagctcactccccccatatattccccctttacatgttttcttataagacatacagtttaatcaattaacaaactaaacagcttatatactggcaatatattacagatgggtttatgtcagagtaatagatcacatgaaatggaccatgtggtaccccagtgcattatgtcttggtagagccctgaggacactgacagtagcatctctaagtaagtagtgctgtatgaatacagacacatgcggatctgtatctacatccatctgactaggccaaggagcaggtagatgcaagatagagacacacacatgctggatggggccactgcacaccttgtcatgccatttaaaagggcagttacaggttgccggttttgcagccattaaaattacactttatggaaaaggcttctctaattgtgtctgatttgctttctgtagtaagcatcattggaagaagaccaaagcaagagcaactagaagttaaatatacatttgagcttagctgcaatacagaaccctggggaagaagcaggctgaaagatttatttaattttaggcttggattctctcccttgctgttttcttgatgttgtgtgtctgcatttgtgtgtgtgtgtgtgtctgcgtgtgtgtgtgttccatcacatcatctcctgaagaacgctgggtttcgcaggcaggcggctagtcacctgcaacaacccaggggtcctgccgaggcttccaggctgctgtcagtgtcagatgccagggtctggtcggtggacatggaggagatgtcattgacagacgaggatggagggagactctcactgctgttcactgctgcacctgaaggagaaggctgtccttttactacaccatttttagtcttttcttctgaattcattacttccttgtagataagttctttccattcttcaattgtgtgttctctttcatccaactgcttgtcatatatctgaggtggaggcgcctccacttcggctgggtcataccagacgttgatgtagggatgctgtaaggcgtcgtccactgatattctttttgctgggtcaatcactagcatctttgacaacaagtccctggcttggctggctttgagtttattgtgctcggagtccgctgggaagagggaatctgggaagagtttggggaaggtgagtcccgcatacttgggccgattctccacatagtttcttactgtgggttgcaatttcttcatgaattctggacatggtgttcctagttgttcaattaccttattccactggtcaatatcgttctccttgtagcccatccccaggatgacctcaggggctctgtaataacgtgtcaccacatatggagtcatcatgaagcttgtgcctgctgtcctggccagtccaaagtccaggattttcaatgtgcaatcagacttgactacaatgttacttggttttaaatccctgtgaataattccagcagaatggaggtgcttaatgccacacaacatttggtacagcaggtaagacattcgctcatggtctaattccatctgaatcacttgacataagttggcatccatcagttccattactaagtaaacatcttggaactcctccagcgttttctggggtgtgaagacatttaataaactaataatgtttttatggttcacacacttcatgaggaccagctcccggtacgctctcttggcatgtgtttggttctgaaagggtctgctgagcttcttaatggccacatttctgtcaaggacagcatcatacgcggcacaaactatgccctgagccccagagccaataggctttagattctggtagcgcttgagaactgtgaaggttgagtctcccacttccacactgtagaactggttgtcaactttgcttttgctcatgttgtaatgtttggcaatatatgacacatccacttgtttatcgaatcccttgttttacctgtaaggaacacacacctgacaaaaggcaattttcacatccaatgttggttcactgcagtagtataagaaatggaggctcataaataccacagcttgtatggtttctcatctataggaaacgggtctaattcaacagtttcttgcataagttgccatagtgaagatctgagatgggcctgctgttggtgtttctcacactagccattccgtgcctgagaactacgatcctgatccggcagtgtttgccccagaaatcctccctacttgtttttcattaaccacattccagactaacatggaagagattctttggagatatggagattgtttaaaattaacgatggacaggtgatttccaagaaaacccaatcttaaactcactcaagcccctaggaattgaggggtgaggacaaaaaaggaaatttgtaaaaatgaaaaaagaaaagaaaaaggtaagcatatagcaagcaccacccacccccataaaaataaaaagtgaaggggaggttaaagaaaatagaagaagagtggcttgctgaatcaccctctttcactgcctggaaaccattgtgcagcgtgatgctgcctgtaccattgtg

SEQ ID NO: 9199 - RNA, 4032 nt, Homo sapiens
  source 1..4032: mol_type = other RNA
agacagtagttcttgcctggtttactctgagggggaaattcaccacttatgcaggtacgagagatagcctgtcaagcactttgaagatgctggctggagacttccttctgtcttgtgatgtcatcttgcggctgatgaaattccccttgagactctctttaaagcagcttcctgctctccgcacttaatcccatgtggtataaagtaagggaggggagaagccacagatatatcaagagaaaagtaccgagaaagaaaatcagtaaagaattagagatacagagaggagaagtttttaaaaaaaaaaaaaaaaaacaggaatatgaaagagagggagctcaagtgactgaggaggcatttttaacaatcaggttatctgcaatattaaccagaaaaaaaatggtagcaaaatagagaaaatgggccatttttattccaggggacaagctgcacaaaggaatgttcttctatttattttaaacaaatgactgcgtgtactgaatctgactgtgtgaaataatctcagaatggcagcaccactggcatggcgatggtgcaggtgggtgcagttccctgtggtctctattgcttgaagagagaaagaaagttccctattattatatttaaggcagttttcagagcactggcattcttgtttgctctgttttggggatattctatttgccaatcagttcacactcatcaaccatccacttcctgtctttcacttcttcaggtgaaatatcaccactctagtgagcaccaacatggtcagagtgcaaataactgtgatggatacttcgaagtgaataagaagggaagcctgattattgctgagatcaccttggtattgccttgtacataaccaagatgtttcacagtgcctccttaagtgctcaggaaagcactttcatttaatttaatttaagctaaattctggagattttgctaaacattgacattaatgcttcatggcttttaagacaaactcatattgctaaaactatttggcagcagtaaatttatgggcagagttattgctcttacatctactgcagtacaaaactcagatgatcagcccttcgattgctcatacttattaaaataaataaataaacatgaaacatcagccacattaaggagtcagggaaactcctgaggaataacaatgtctctggagatgttttcaaatgctaacctgagactcacactgtggtttgggggtttcattattattattattattttatttcagaagaggaaagtaatattatttctcaaaataaaactttggcagagtatgaatcagggaagcagcccacacatggaaaacacaatccacaatctgaaagtagtctaggcaggctcatttttttgttgaaggaattcacatggaggcaattctgctcagttccagagagagattcttatcatcaaaagcacacacaataaccttgcttcaccacctgccactttctccagtggcctcttgttgtgaccagtaattgagaaatgacaaatgggtatagagccaaatctctaaaacagggacaccagtgtctcctagtatctgggtaataacctcctttcagtcttagtccacaccacacactaccctccagtctctcctactctttactgtcacagaaaagactctcagcttttattcacacctgccttcagaaggccaaaccattttgtgcctgaaaactgttacccactcgccccacactttacataagtatcacatatgttctttctacaaattggtatacaggtgccatttaatccattcaaatttggaagctacatcttcaagggtctgagagagctcactccccccatatattccccctttacatgttttcttataagacatacagtttaatcaattaacaaactaaacagcttatatactggcaatatattacagatgggtttatgtcagagtaatagatcacatgaaatggaccatgtggtaccccagtgcattatgtcttggtagagccctgaggacactgacagtagcatctctaagtaagtagtgctgtatgaatacagacacatgcggatctgtatctacatccatctgactaggccaaggagcaggtagatgcaagatagagacacacacatgctggatggggccactgcacaccttgtcatgccatttaaaagggcagttacaggttgccggttttgcagccattaaaattacactttatggaaaaggcttctctaattgtgtctgatttgctttctgtagtaagcatcattggaagaagaccaaagcaagagcaactagaagttaaatatacatttgagcttagctgcaatacagaaccctggggaagaagcaggctgaaagatttatttaattttaggcttggattctctcccttgctgttttcttgatgttgtgtgtctgcatttgtgtgtgtgtgtgtgtctgcgtgtgtgtgtgttccatcacatcatctcctgaagaacgctgggtttcgcaggcaggcggctagtcacctgcaacaacccaggggtcctgccgaggcttccaggctgctgtcagtgtcagatgccagggtctggtcggtggacatggaggagatgtcattgacagacgaggatggagggagactctcactgctgttcactgctgcacctgaaggagaaggctgtccttttactacaccatttttagtcttttcttctgaattcattacttccttgtagataagttctttccattcttcaattgtgtgttctctttcatccaactgcttgtcatatatctgaggtggaggcgcctccacttcggctgggtcataccagacgttgatgtagggatgctgtaaggcgtcgtccactgatattctttttgctgggtcaatcactagcatctttgacaacaagtccctggcttggctggctttgagtttattgtgctcggagtccgctgggaagagggaatctgggaagagtttggggaaggtgagtcccgcatacttgggccgattctccacatagtttcttactgtgggttgcaatttcttcatgaattctggacatggtgttcctagttgttcaattaccttattccactggtcaatatgatcagtgccaggaaacagcactgcaccttttatcatttctcccatgatgcaccctactgaccacatgtcaacgttctccttgtagcccatccccaggatgacctcaggggctctgtaataacgtgtcaccacatatggagtcatcatgaagcttgtgcctgctgtcctggccagtccaaagtccaggattttcaatgtgcaatcagacttgactacaatgttacttggttttaaatccctgtgaataattccagcagaatggaggtgcttaatgccacacaacatttggtacagcaggtaagacattcgctcatggtctaattccatctgaatcacttgacataagttggcatccatcagttccattactaagtaaacatcttggaactcctccagcgttttctggggtgtgaagacatttaataaactaataatgtttttatggttcacacacttcatgaggaccagctcccggtacgctctcttggcatgtgtttggttctgaaagggtctgctgagcttcttaatggccacatttctgtcaaggacagcatcatacgcggcacaaactatgccctgagccccagagccaataggctttagattctggtagcgcttgagaactgtgaaggttgagtctcccacttccacactgtagaactggttgtcaactttgcttttgctcatgttgtaatgtttggcaatatatgacacatccacttgtttatcgaatccctgacaaaaggcaattttcacatccaatgttggttcactgcagtagtataagaaatggaggctcataaataccacagcttgtatggtttctcatctataggaaacgggtctaattcaacagtttcttgcataagttgccatagtgaagatctgagatgggcctgctgttggtgtttctcacactagc

SEQ ID NO: 9200 - RNA, 4435 nt, Homo sapiens
  source 1..4435: mol_type = other RNA
agacagtagttcttgcctggtttactctgagggggaaattcaccacttatgcaggtacgagagatagcctgtcaagcactttgaagatgctggctggagacttccttctgtcttgtgatgtcatcttgcggctgatgaaattccccttgagactctctttaaagcagcttcctgctctccgcacttaatcccatgtggtataaagtaagggaggggagaagccacagatatatcaagagaaaagtaccgagaaagaaaatcagtaaagaattagagatacagagaggagaagtttttaaaaaaaaaaaaaaaaaacaggaatatgaaagagagggagctcaagtgactgaggaggcatttttaacaatcaggttatctgcaatattaaccagaaaaaaaatggtagcaaaatagagaaaatgggccatttttattccaggggacaagctgcacaaaggaatgttcttctatttattttaaacaaatgactgcgtgtactgaatctgactgtgtgaaataatctcagaatggcagcaccactggcatggcgatggtgcaggtgggtgcagttccctgtggtctctattgcttgaagagagaaagaaagttccctattattatatttaaggcagttttcagagcactggcattcttgtttgctctgttttggggatattctatttgccaatcagttcacactcatcaaccatccacttcctgtctttcacttcttcaggtgaaatatcaccactctagtgagcaccaacatggtcagagtgcaaataactgtgatggatacttcgaagtgaataagaagggaagcctgattattgctgagatcaccttggtattgccttgtacataaccaagatgtttcacagtgcctccttaagtgctcaggaaagcactttcatttaatttaatttaagctaaattctggagattttgctaaacattgacattaatgcttcatggcttttaagacaaactcatattgctaaaactatttggcagcagtaaatttatgggcagagttattgctcttacatctactgcagtacaaaactcagatgatcagcccttcgattgctcatacttattaaaataaataaataaacatgaaacatcagccacattaaggagtcagggaaactcctgaggaataacaatgtctctggagatgttttcaaatgctaacctgagactcacactgtggtttgggggtttcattattattattattattttatttcagaagaggaaagtaatattatttctcaaaataaaactttggcagagtatgaatcagggaagcagcccacacatggaaaacacaatccacaatctgaaagtagtctaggcaggctcatttttttgttgaaggaattcacatggaggcaattctgctcagttccagagagagattcttatcatcaaaagcacacacaataaccttgcttcaccacctgccactttctccagtggcctcttgttgtgaccagtaattgagaaatgacaaatgggtatagagccaaatctctaaaacagggacaccagtgtctcctagtatctgggtaataacctcctttcagtcttagtccacaccacacactaccctccagtctctcctactctttactgtcacagaaaagactctcagcttttattcacacctgccttcagaaggccaaaccattttgtgcctgaaaactgttacccactcgccccacactttacataagtatcacatatgttctttctacaaattggtatacaggtgccatttaatccattcaaatttggaagctacatcttcaagggtctgagagagctcactccccccatatattccccctttacatgttttcttataagacatacagtttaatcaattaacaaactaaacagcttatatactggcaatatattacagatgggtttatgtcagagtaatagatcacatgaaatggaccatgtggtaccccagtgcattatgtcttggtagagccctgaggacactgacagtagcatctctaagtaagtagtgctgtatgaatacagacacatgcggatctgtatctacatccatctgactaggccaaggagcaggtagatgcaagatagagacacacacatgctggatggggccactgcacaccttgtcatgccatttaaaagggcagttacaggttgccggttttgcagccattaaaattacactttatggaaaaggcttctctaattgtgtctgatttgctttctgtagtaagcatcattggaagaagaccaaagcaagagcaactagaagttaaatatacatttgagcttagctgcaatacagaaccctggggaagaagcaggctgaaagatttatttaattttaggcttggattctctcccttgctgttttcttgatgttgtgtgtctgcatttgtgtgtgtgtgtgtgtctgcgtgtgtgtgtgttccatcacatcatctcctgaagaacgctgggtttcgcaggcaggcggctagtcacctgcaacaacccaggggtcctgccgaggcttccaggctgctgtcagtgtcagatgccagggtctggtcggtggacatggaggagatgtcattgacagacgaggatggagggagactctcactgctgttcactgctgcacctgaaggagaaggctgtccttttactacaccatttttagtcttttcttctgaattcattacttccttgtagataagttctttccattcttcaattgtgtgttctctttcatccaactgcttgtcatatatctgaggtggaggcgcctccacttcggctgggtcataccagacgttgatgtagggatgctgtaaggcgtcgtccactgatattctttttgctgggtcaatcactagcatctttgacaacaagtccctggcttggctggctttgagtttattgtgctcggagtccgctgggaagagggaatctgggaagagtttggggaaggtgagtcccgcatacttgggccgattctccacatagtttcttactgtgggttgcaatttcttcatgaattctggacatggtgttcctagttgttcaattaccttattccactggtcaatatgatcagtgccaggaaacagcactgcaccttttatcatttctcccatgatgcaccctactgaccacatgtcaacgttctccttgtagcccatccccaggatgacctcaggggctctgtaataacgtgtcaccacatatggagtcatcatgaagcttgtgcctgctgtcctggccagtccaaagtccaggattttcaatgtgcaatcagacttgactacaatgttacttggttttaaatccctgtgaataattccagcagaatggaggtgcttaatgccacacaacatttggtacagcaggtaagacattcgctcatggtctaattccatctgaatcacttgacataagttggcatccatcagttccattactaagtaaacatcttggaactcctccagcgttttctggggtgtgaagacatttaataaactaataatgtttttatggttcacacacttcatgaggaccagctcccggtacgctctcttggcatgtgtttggttctgaaagggtctgctgagcttcttaatggccacatttctgtcaaggacagcatcatacgcggcacaaactatgccctgagccccagagccaataggctttagattctggtagcgcttgagaactgtgaaggttgagtctcccacttccacactgtagaactggttgtcaactttgcttttgctcatgttgtaatgtttggcaatatatgacacatccacttgtttatcgaatccctgacaaaaggcaattttcacatccaatgttggttcactgcagtagtataagaaatggaggctcataaataccacagcttgtatggtttctcatctataggaaacgggtctaattcaacagtttcttgcataagttgccatagtgaagatctgagatgggcctgctgttggtgtttctcacactagccattccgtgcctgagaactacgatcctgatccggcagtgtttgccccagaaatcctccctacttgtttttcattaaccacattccagactaacatggaagagattctttggagatatggagattgtttaaaattaacgatggacaggtgatttccaagaaaacccaatcttaaactcactcaagcccctaggaattgaggggtgaggacaaaaaaggaaatttgtaaaaatgaaaaaagaaaagaaaaaggtaagcatatagcaagcaccacccacccccataaaaataaaaagtgaaggggaggttaaagaaaatagaagaagagtggcttgctgaatcaccctctttcactgcctggaaaccattgtgcagcgtgatgctgcctgtaccattgtggaacct

SEQ ID NO: 9201 - RNA, 4456 nt, Homo sapiens
  source 1..4456: mol_type = other RNA
agacagtagttcttgcctggtttactctgagggggaaattcaccacttatgcaggtacgagagatagcctgtcaagcactttgaagatgctggctggagacttccttctgtcttgtgatgtcatcttgcggctgatgaaattccccttgagactctctttaaagcagcttcctgctctccgcacttaatcccatgtggtataaagtaagggaggggagaagccacagatatatcaagagaaaagtaccgagaaagaaaatcagtaaagaattagagatacagagaggagaagtttttaaaaaaaaaaaaaaaaaacaggaatatgaaagagagggagctcaagtgactgaggaggcatttttaacaatcaggttatctgcaatattaaccagaaaaaaaatggtagcaaaatagagaaaatgggccatttttattccaggggacaagctgcacaaaggaatgttcttctatttattttaaacaaatgactgcgtgtactgaatctgactgtgtgaaataatctcagaatggcagcaccactggcatggcgatggtgcaggtgggtgcagttccctgtggtctctattgcttgaagagagaaagaaagttccctattattatatttaaggcagttttcagagcactggcattcttgtttgctctgttttggggatattctatttgccaatcagttcacactcatcaaccatccacttcctgtctttcacttcttcaggtgaaatatcaccactctagtgagcaccaacatggtcagagtgcaaataactgtgatggatacttcgaagtgaataagaagggaagcctgattattgctgagatcaccttggtattgccttgtacataaccaagatgtttcacagtgcctccttaagtgctcaggaaagcactttcatttaatttaatttaagctaaattctggagattttgctaaacattgacattaatgcttcatggcttttaagacaaactcatattgctaaaactatttggcagcagtaaatttatgggcagagttattgctcttacatctactgcagtacaaaactcagatgatcagcccttcgattgctcatacttattaaaataaataaataaacatgaaacatcagccacattaaggagtcagggaaactcctgaggaataacaatgtctctggagatgttttcaaatgctaacctgagactcacactgtggtttgggggtttcattattattattattattttatttcagaagaggaaagtaatattatttctcaaaataaaactttggcagagtatgaatcagggaagcagcccacacatggaaaacacaatccacaatctgaaagtagtctaggcaggctcatttttttgttgaaggaattcacatggaggcaattctgctcagttccagagagagattcttatcatcaaaagcacacacaataaccttgcttcaccacctgccactttctccagtggcctcttgttgtgaccagtaattgagaaatgacaaatgggtatagagccaaatctctaaaacagggacaccagtgtctcctagtatctgggtaataacctcctttcagtcttagtccacaccacacactaccctccagtctctcctactctttactgtcacagaaaagactctcagcttttattcacacctgccttcagaaggccaaaccattttgtgcctgaaaactgttacccactcgccccacactttacataagtatcacatatgttctttctacaaattggtatacaggtgccatttaatccattcaaatttggaagctacatcttcaagggtctgagagagctcactccccccatatattccccctttacatgttttcttataagacatacagtttaatcaattaacaaactaaacagcttatatactggcaatatattacagatgggtttatgtcagagtaatagatcacatgaaatggaccatgtggtaccccagtgcattatgtcttggtagagccctgaggacactgacagtagcatctctaagtaagtagtgctgtatgaatacagacacatgcggatctgtatctacatccatctgactaggccaaggagcaggtagatgcaagatagagacacacacatgctggatggggccactgcacaccttgtcatgccatttaaaagggcagttacaggttgccggttttgcagccattaaaattacactttatggaaaaggcttctctaattgtgtctgatttgctttctgtagtaagcatcattggaagaagaccaaagcaagagcaactagaagttaaatatacatttgagcttagctgcaatacagaaccctggggaagaagcaggctgaaagatttatttaattttaggcttggattctctcccttgctgttttcttgatgttgtgtgtctgcatttgtgtgtgtgtgtgtgtctgcgtgtgtgtgtgttccatcacatcatctcctgaagaacgctgggtttcgcaggcaggcggctagtcacctgcaacaacccaggggtcctgccgaggcttccaggctgctgtcagtgtcagatgccagggtctggtcggtggacatggaggagatgtcattgacagacgaggatggagggagactctcactgctgttcactgctgcacctgaaggagaaggctgtccttttactacaccatttttagtcttttcttctgaattcattacttccttgtagataagttctttccattcttcaattgtgtgttctctttcatccaactgcttgtcatatatctgaggtggaggcgcctccacttcggctgggtcataccagacgttgatgtagggatgctgtaaggcgtcgtccactgatattctttttgctgggtcaatcactagcatctttgacaacaagtccctggcttggctggctttgagtttattgtgctcggagtccgctgggaagagggaatctgggaagagtttggggaaggtgagtcccgcatacttgggccgattctccacatagtttcttactgtgggttgcaatttcttcatgaattctggacatggtgttcctagttgttcaattaccttattccactggtcaatatgatcagtgccaggaaacagcactgcaccttttatcatttctcccatgatgcaccctactgaccacatgtcaacgttctccttgtagcccatccccaggatgacctcaggggctctgtaataacgtgtcaccacatatggagtcatcatgaagcttgtgcctgctgtcctggccagtccaaagtccaggattttcaatgtgcaatcagacttgactacaatgttacttggttttaaatccctgtgaataattccagcagaatggaggtgcttaatgccacacaacatttggtacagcaggtaagacattcgctcatggtctaattccatctgaatcacttgacataagttggcatccatcagttccattactaagtaaacatcttggaactcctccagcgttttctggggtgtgaagacatttaataaactaataatgtttttatggttcacacacttcatgaggaccagctcccggtacgctctcttggcatgtgtttggttctgaaagggtctgctgagcttcttaatggccacatttctgtcaaggacagcatcatacgcggcacaaactatgccctgagccccagagccaataggctttagattctggtagcgcttgagaactgtgaaggttgagtctcccacttccacactgtagaactggttgtcaactttgcttttgctcatgttgtaatgtttggcaatatatgacacatccacttgtttatcgaatcccttgttttacctgtaaggaacacacacctgacaaaaggcaattttcacatccaatgttggttcactgcagtagtataagaaatggaggctcataaataccacagcttgtatggtttctcatctataggaaacgggtctaattcaacagtttcttgcataagttgccatagtgaagatctgagatgggcctgctgttggtgtttctcacactagccattccgtgcctgagaactacgatcctgatccggcagtgtttgccccagaaatcctccctacttgtttttcattaaccacattccagactaacatggaagagattctttggagatatggagattgtttaaaattaacgatggacaggtgatttccaagaaaacccaatcttaaactcactcaagcccctaggaattgaggggtgaggacaaaaaaggaaatttgtaaaaatgaaaaaagaaaagaaaaaggtaagcatatagcaagcaccacccacccccataaaaataaaaagtgaaggggaggttaaagaaaatagaagaagagtggcttgctgaatcaccctctttcactgcctggaaaccattgtgcagcgtgatgctgcctgtaccattgtg

SEQ ID NO: 9202 - RNA, 4260 nt, Homo sapiens
  source 1..4260: mol_type = other RNA
agacagtagttcttgcctggtttactctgagggggaaattcaccacttatgcaggtacgagagatagcctgtcaagcactttgaagatgctggctggagacttccttctgtcttgtgatgtcatcttgcggctgatgaaattccccttgagactctctttaaagcagcttcctgctctccgcacttaatcccatgtggtataaagtaagggaggggagaagccacagatatatcaagagaaaagtaccgagaaagaaaatcagtaaagaattagagatacagagaggagaagtttttaaaaaaaaaaaaaaaaaacaggaatatgaaagagagggagctcaagtgactgaggaggcatttttaacaatcaggttatctgcaatattaaccagaaaaaaaatggtagcaaaatagagaaaatgggccatttttattccaggggacaagctgcacaaaggaatgttcttctatttattttaaacaaatgactgcgtgtactgaatctgactgtgtgaaataatctcagaatggcagcaccactggcatggcgatggtgcaggtgggtgcagttccctgtggtctctattgcttgaagagagaaagaaagttccctattattatatttaaggcagttttcagagcactggcattcttgtttgctctgttttggggatattctatttgccaatcagttcacactcatcaaccatccacttcctgtctttcacttcttcaggtgaaatatcaccactctagtgagcaccaacatggtcagagtgcaaataactgtgatggatacttcgaagtgaataagaagggaagcctgattattgctgagatcaccttggtattgccttgtacataaccaagatgtttcacagtgcctccttaagtgctcaggaaagcactttcatttaatttaatttaagctaaattctggagattttgctaaacattgacattaatgcttcatggcttttaagacaaactcatattgctaaaactatttggcagcagtaaatttatgggcagagttattgctcttacatctactgcagtacaaaactcagatgatcagcccttcgattgctcatacttattaaaataaataaataaacatgaaacatcagccacattaaggagtcagggaaactcctgaggaataacaatgtctctggagatgttttcaaatgctaacctgagactcacactgtggtttgggggtttcattattattattattattttatttcagaagaggaaagtaatattatttctcaaaataaaactttggcagagtatgaatcagggaagcagcccacacatggaaaacacaatccacaatctgaaagtagtctaggcaggctcatttttttgttgaaggaattcacatggaggcaattctgctcagttccagagagagattcttatcatcaaaagcacacacaataaccttgcttcaccacctgccactttctccagtggcctcttgttgtgaccagtaattgagaaatgacaaatgggtatagagccaaatctctaaaacagggacaccagtgtctcctagtatctgggtaataacctcctttcagtcttagtccacaccacacactaccctccagtctctcctactctttactgtcacagaaaagactctcagcttttattcacacctgccttcagaaggccaaaccattttgtgcctgaaaactgttacccactcgccccacactttacataagtatcacatatgttctttctacaaattggtatacaggtgccatttaatccattcaaatttggaagctacatcttcaagggtctgagagagctcactccccccatatattccccctttacatgttttcttataagacatacagtttaatcaattaacaaactaaacagcttatatactggcaatatattacagatgggtttatgtcagagtaatagatcacatgaaatggaccatgtggtaccccagtgcattatgtcttggtagagccctgaggacactgacagtagcatctctaagtaagtagtgctgtatgaatacagacacatgcggatctgtatctacatccatctgactaggccaaggagcaggtagatgcaagatagagacacacacatgctggatggggccactgcacaccttgtcatgccatttaaaagggcagttacaggttgccggttttgcagccattaaaattacactttatggaaaaggcttctctaattgtgtctgatttgctttctgtagtaagcatcattggaagaagaccaaagcaagagcaactagaagttaaatatacatttgagcttagctgcaatacagaaccctggggaagaagcaggctgaaagatttatttaattttaggcttggattctctcccttgctgttttcttgatgttgtgtgtctgcatttgtgtgtgtgtgtgtgtctgcgtgtgtgtgtgttccatcacatcatctcctgaagaacgctgggtttcgcaggcaggcggctagtcacctgcaacaacccaggggtcctgccgaggcttccaggctgctgtcagtgtcagatgccagggtctggtcggtggacatggaggagatgtcattgacagacgaggatggagggagactctcactgctgttcactgctgcacctgaaggagaaggctgtccttttactacaccatttttagtcttttcttctgaattcattacttccttgtagataagttctttccattcttcaattgtgtgttctctttcatccaactgcttgtcatatatctgaggtggaggcgcctccacttcggctgggtcataccagacgttgatgtagggatgctgtaaggcgtcgtccactgatattctttttgctgggtcaatcactagcatctttgacaacaagtccctggcttggctggctttgagtttattgtgctcggagtccgctgggaagagggaatctgggaagagtttggggaaggtgagtcccgcatacttgggccgattctccacatagtttcttactgtgggttgcaatttcttcatgaattctggacatggtgttcctagttgttcaattaccttattccactggtcaatatgatcagtgccaggaaacagcactgcaccttttatcatttctcccatgatgcaccctactgaccacatgtcaacgttctccttgtagcccatccccaggatgacctcaggggctctgtaataacgtgtcaccacatatggagtcatcatgaagcttgtgcctgctgtcctggccagtccaaagtccaggattttcaatgtgcaatcagacttgactacaatgttacttggttttaaatccctgtgaataattccagcagaatggaggtgcttaatgccacacaacatttggtacagcaggtaagacattcgctcatggtctaattccatctgaatcacttgacataagttggcatccatcagttccattactaagtaaacatcttggaactcctccagcgttttctggggtgtgaagacatttaataaactaataatgtttttatggttcacacacttcatgaggaccagctcccggtacgctctcttggcatgtgtttggttctgaaagggtctgctgagcttcttaatggccacatttctgtcaaggacagcatcatacgcggcacaaactatgccctgagccccagagccaataggctttagattctggtagcgcttgagaactgtgaaggttgagtctcccacttccacactgtagaactggttgtcaactttgcttttgctcatgttgtaatgtttggcaatatatgacacatccacttgtttatcgaatcccttgttttacctgtaaggaacacacacctgacaaaaggcaattttcacatccaatgttggttcactgcagtagtataagaaatggaggctcataaataccacagcttgtatggtttctcatctataggaaacgggtctaattcaacagtttcttgcataagttgccatagtgaagatctgagatgggcctgctgttggtgtttctcacactagcgcatttttcactctcctcctcactccctagggtcatagttttgattctgaagttagaagtgtgggggtcgtcggctgcattttcaacttggcctaaaagttggagttcaccacactgcaggcgctaggaactctgccgctcggtcaccaacctgagcctctggctagtccgaagaacgcgaaaagccaggcccaaggcact

SEQ ID NO: 9203 - RNA, 4370 nt, Homo sapiens
  source 1..4370: mol_type = other RNA
agacagtagttcttgcctggtttactctgagggggaaattcaccacttatgcaggtacgagagatagcctgtcaagcactttgaagatgctggctggagacttccttctgtcttgtgatgtcatcttgcggctgatgaaattccccttgagactctctttaaagcagcttcctgctctccgcacttaatcccatgtggtataaagtaagggaggggagaagccacagatatatcaagagaaaagtaccgagaaagaaaatcagtaaagaattagagatacagagaggagaagtttttaaaaaaaaaaaaaaaaaacaggaatatgaaagagagggagctcaagtgactgaggaggcatttttaacaatcaggttatctgcaatattaaccagaaaaaaaatggtagcaaaatagagaaaatgggccatttttattccaggggacaagctgcacaaaggaatgttcttctatttattttaaacaaatgactgcgtgtactgaatctgactgtgtgaaataatctcagaatggcagcaccactggcatggcgatggtgcaggtgggtgcagttccctgtggtctctattgcttgaagagagaaagaaagttccctattattatatttaaggcagttttcagagcactggcattcttgtttgctctgttttggggatattctatttgccaatcagttcacactcatcaaccatccacttcctgtctttcacttcttcaggtgaaatatcaccactctagtgagcaccaacatggtcagagtgcaaataactgtgatggatacttcgaagtgaataagaagggaagcctgattattgctgagatcaccttggtattgccttgtacataaccaagatgtttcacagtgcctccttaagtgctcaggaaagcactttcatttaatttaatttaagctaaattctggagattttgctaaacattgacattaatgcttcatggcttttaagacaaactcatattgctaaaactatttggcagcagtaaatttatgggcagagttattgctcttacatctactgcagtacaaaactcagatgatcagcccttcgattgctcatacttattaaaataaataaataaacatgaaacatcagccacattaaggagtcagggaaactcctgaggaataacaatgtctctggagatgttttcaaatgctaacctgagactcacactgtggtttgggggtttcattattattattattattttatttcagaagaggaaagtaatattatttctcaaaataaaactttggcagagtatgaatcagggaagcagcccacacatggaaaacacaatccacaatctgaaagtagtctaggcaggctcatttttttgttgaaggaattcacatggaggcaattctgctcagttccagagagagattcttatcatcaaaagcacacacaataaccttgcttcaccacctgccactttctccagtggcctcttgttgtgaccagtaattgagaaatgacaaatgggtatagagccaaatctctaaaacagggacaccagtgtctcctagtatctgggtaataacctcctttcagtcttagtccacaccacacactaccctccagtctctcctactctttactgtcacagaaaagactctcagcttttattcacacctgccttcagaaggccaaaccattttgtgcctgaaaactgttacccactcgccccacactttacataagtatcacatatgttctttctacaaattggtatacaggtgccatttaatccattcaaatttggaagctacatcttcaagggtctgagagagctcactccccccatatattccccctttacatgttttcttataagacatacagtttaatcaattaacaaactaaacagcttatatactggcaatatattacagatgggtttatgtcagagtaatagatcacatgaaatggaccatgtggtaccccagtgcattatgtcttggtagagccctgaggacactgacagtagcatctctaagtaagtagtgctgtatgaatacagacacatgcggatctgtatctacatccatctgactaggccaaggagcaggtagatgcaagatagagacacacacatgctggatggggccactgcacaccttgtcatgccatttaaaagggcagttacaggttgccggttttgcagccattaaaattacactttatggaaaaggcttctctaattgtgtctgatttgctttctgtagtaagcatcattggaagaagaccaaagcaagagcaactagaagttaaatatacatttgagcttagctgcaatacagaaccctggggaagaagcaggctgaaagatttatttaattttaggcttggattctctcccttgctgttttcttgatgttgtgtgtctgcatttgtgtgtgtgtgtgtgtctgcgtgtgtgtgtgttccatcacatcatctcctgaagaacgctgggtttcgcaggcaggcggctagtcacctgcaacaacccaggggtcctgccgaggcttccaggctgctgtcagtgtcagatgccagggtctggtcggtggacatggaggagatgtcattgacagacgaggatggagggagactctcactgctgttcactgctgcacctgaaggagaaggctgtccttttactacaccatttttagtcttttcttctgaattcattacttccttgtagataagttctttccattcttcaattgtgtgttctctttcatccaactgcttgtcatatatctgaggtggaggcgcctccacttcggctgggtcataccagacgttgatgtagggatgctgtaaggcgtcgtccactgatattctttttgctgggtcaatcactagcatctttgacaacaagtccctggcttggctggctttgagtttattgtgctcggagtccgctgggaagagggaatctgggaagagtttggggaaggtgagtcccgcatacttgggccgattctccacatagtttcttactgtgggttgcaatttcttcatgaattctggacatggtgttcctagttgttcaattaccttattccactggtcaatatgatcagtgccaggaaacagcactgcaccttttatcatttctcccatgatgcaccctactgaccacatgtcaacgttctccttgtagcccatccccaggatgacctcaggggctctgtaataacgtgtcaccacatatggagtcatcatgaagcttgtgcctgctgtcctggccagtccaaagtccaggattttcaatgtgcaatcagacttgactacaatgttacttggttttaaatccctgtgaataattccagcagaatggaggtgcttaatgccacacaacatttggtacagcaggtaagacattcgctcatggtctaattccatctgaatcacttgacataagttggcatccatcagttccattactaagtaagtttttatggttcacacacttcatgaggaccagctcccggtacgctctcttggcatgtgtttggttctgaaagggtctgctgagcttcttaatggccacatttctgtcaaggacagcatcatacgcggcacaaactatgccctgagccccagagccaataggctttagattctggtagcgcttgagaactgtgaaggttgagtctcccacttccacactgtagaactggttgtcaactttgcttttgctcatgttgtaatgtttggcaatatatgacacatccacttgtttatcgaatccctgacaaaaggcaattttcacatccaatgttggttcactgcagtagtataagaaatggaggctcataaataccacagcttgtatggtttctcatctataggaaacgggtctaattcaacagtttcttgcataagttgccatagtgaagatctgagatgggcctgctgttggtgtttctcacactagccattccgtgcctgagaactacgatcctgatccggcagtgtttgccccagaaatcctccctacttgtttttcattaaccacattccagactaacatggaagagattctttggagatatggagattgtttaaaattaacgatggacaggtgatttccaagaaaacccaatcttaaactcactcaagcccctaggaattgaggggtgaggacaaaaaaggaaatttgtaaaaatgaaaaaagaaaagaaaaaggtaagcatatagcaagcaccacccacccccataaaaataaaaagtgaaggggaggttaaagaaaatagaagaagagtggcttgctgaatcaccctctttcactgcctggaaaccattgtgcagcgtgatgctgcctgtaccattgtg

SEQ ID NO: 9204 - RNA, 4127 nt, Homo sapiens
  source 1..4127: mol_type = other RNA
agacagtagttcttgcctggtttactctgagggggaaattcaccacttatgcaggtacgagagatagcctgtcaagcactttgaagatgctggctggagacttccttctgtcttgtgatgtcatcttgcggctgatgaaattccccttgagactctctttaaagcagcttcctgctctccgcacttaatcccatgtggtataaagtaagggaggggagaagccacagatatatcaagagaaaagtaccgagaaagaaaatcagtaaagaattagagatacagagaggagaagtttttaaaaaaaaaaaaaaaaaacaggaatatgaaagagagggagctcaagtgactgaggaggcatttttaacaatcaggttatctgcaatattaaccagaaaaaaaatggtagcaaaatagagaaaatgggccatttttattccaggggacaagctgcacaaaggaatgttcttctatttattttaaacaaatgactgcgtgtactgaatctgactgtgtgaaataatctcagaatggcagcaccactggcatggcgatggtgcaggtgggtgcagttccctgtggtctctattgcttgaagagagaaagaaagttccctattattatatttaaggcagttttcagagcactggcattcttgtttgctctgttttggggatattctatttgccaatcagttcacactcatcaaccatccacttcctgtctttcacttcttcaggtgaaatatcaccactctagtgagcaccaacatggtcagagtgcaaataactgtgatggatacttcgaagtgaataagaagggaagcctgattattgctgagatcaccttggtattgccttgtacataaccaagatgtttcacagtgcctccttaagtgctcaggaaagcactttcatttaatttaatttaagctaaattctggagattttgctaaacattgacattaatgcttcatggcttttaagacaaactcatattgctaaaactatttggcagcagtaaatttatgggcagagttattgctcttacatctactgcagtacaaaactcagatgatcagcccttcgattgctcatacttattaaaataaataaataaacatgaaacatcagccacattaaggagtcagggaaactcctgaggaataacaatgtctctggagatgttttcaaatgctaacctgagactcacactgtggtttgggggtttcattattattattattattttatttcagaagaggaaagtaatattatttctcaaaataaaactttggcagagtatgaatcagggaagcagcccacacatggaaaacacaatccacaatctgaaagtagtctaggcaggctcatttttttgttgaaggaattcacatggaggcaattctgctcagttccagagagagattcttatcatcaaaagcacacacaataaccttgcttcaccacctgccactttctccagtggcctcttgttgtgaccagtaattgagaaatgacaaatgggtatagagccaaatctctaaaacagggacaccagtgtctcctagtatctgggtaataacctcctttcagtcttagtccacaccacacactaccctccagtctctcctactctttactgtcacagaaaagactctcagcttttattcacacctgccttcagaaggccaaaccattttgtgcctgaaaactgttacccactcgccccacactttacataagtatcacatatgttctttctacaaattggtatacaggtgccatttaatccattcaaatttggaagctacatcttcaagggtctgagagagctcactccccccatatattccccctttacatgttttcttataagacatacagtttaatcaattaacaaactaaacagcttatatactggcaatatattacagatgggtttatgtcagagtaatagatcacatgaaatggaccatgtggtaccccagtgcattatgtcttggtagagccctgaggacactgacagtagcatctctaagtaagtagtgctgtatgaatacagacacatgcggatctgtatctacatccatctgactaggccaaggagcaggtagatgcaagatagagacacacacatgctggatggggccactgcacaccttgtcatgccatttaaaagggcagttacaggttgccggttttgcagccattaaaattacactttatggaaaaggcttctctaattgtgtctgatttgctttctgtagtaagcatcattggaagaagaccaaagcaagagcaactagaagttaaatatacatttgagcttagctgcaatacagaaccctggggaagaagcaggctgaaagatttatttaattttaggcttggattctctcccttgctgttttcttgatgttgtgtgtctgcatttgtgtgtgtgtgtgtgtctgcgtgtgtgtgtgttccatcacatcatctcctgaagaacgctgggtttcgcaggcaggcggctagtcacctgcaacaacccaggggtcctgccgaggcttccaggctgctgtcagtgtcagatgccagggtctggtcggtggacatggaggagatgtcattgacagacgaggatggagggagactctcactgctgttcactgctgcacctgaaggagaaggctgtccttttactacaccatttttagtcttttcttctgaattcattacttccttgtagataagttctttccattcttcaattgtgtgttctctttcatccaactgcttgtcatatatctgaggtggaggcgcctccacttcggctgggtcataccagacgttgatgtagggatgctgtaaggcgtcgtccactgatattctttttgctgggtcaatcactagcatctttgacaacaagtccctggcttggctggctttgagtttattgtgctcggagtccgctgggaagagggaatctgggaagagtttggggaaggtgagtcccgcatacttgggccgattctccacatagtttcttactgtgggttgcaatttcttcatgaattctggacatggtgttcctagttgttcaattaccttattccactggtcaatatgatcagtgccaggaaacagcactgcaccttttatcatttctcccatgatgcaccctactgaccacatgtcaacgttctccttgtagcccatccccaggatgacctcaggggctctgtaataacgtgtcaccacatatggagtcatcatgaagcttgtgcctgctgtcctggccagtccaaagtccaggattttcaatgtgcaatcagacttgactacaatgttacttggttttaaatccctgtgaataattccagcagaatggaggtgcttaatgccacacaacatttggtacagcaggtaagacattcgctcatggtctaattccatctgaatcacttgacataagttggcatccatcagttccattactaagtaagtttttatggttcacacacttcatgaggaccagctcccggtacgctctcttggcatgtgtttggttctgaaagggtctgctgagcttcttaatggccacatttctgtcaaggacagcatcatacgcggcacaaactatgccctgagccccagagccaataggctttagattctggtagcgcttgagaactgtgaaggttgagtctcccacttccacactgtagaactggttgtcaactttgcttttgctcatgttgtaatgtttggcaatatatgacacatccacttgtttatcgaatccctgacaaaaggcaattttcacatccaatgttggttcactgcagtagtataagaaatggaggctcataaataccacagcttgtatggtttctcatctataggaaacgggtctaattcaacagtttcttgcataagttgccatagtgaagatctgagatgggcctgctgttggtgtttctcacactagccttgggaagaagcatagtcaaataaaaatggaaaccttagtctcagttccactgtgactatgactacccatcagatgttgggcagatagtggctctgtcgacatgtttcttcatctacaatgtatcaggtctagatcacatgataattatggtt

SEQ ID NO: 9205 - RNA, 4238 nt, Homo sapiens
  source 1..4238: mol_type = other RNA
agacagtagttcttgcctggtttactctgagggggaaattcaccacttatgcaggtacgagagatagcctgtcaagcactttgaagatgctggctggagacttccttctgtcttgtgatgtcatcttgcggctgatgaaattccccttgagactctctttaaagcagcttcctgctctccgcacttaatcccatgtggtataaagtaagggaggggagaagccacagatatatcaagagaaaagtaccgagaaagaaaatcagtaaagaattagagatacagagaggagaagtttttaaaaaaaaaaaaaaaaaacaggaatatgaaagagagggagctcaagtgactgaggaggcatttttaacaatcaggttatctgcaatattaaccagaaaaaaaatggtagcaaaatagagaaaatgggccatttttattccaggggacaagctgcacaaaggaatgttcttctatttattttaaacaaatgactgcgtgtactgaatctgactgtgtgaaataatctcagaatggcagcaccactggcatggcgatggtgcaggtgggtgcagttccctgtggtctctattgcttgaagagagaaagaaagttccctattattatatttaaggcagttttcagagcactggcattcttgtttgctctgttttggggatattctatttgccaatcagttcacactcatcaaccatccacttcctgtctttcacttcttcaggtgaaatatcaccactctagtgagcaccaacatggtcagagtgcaaataactgtgatggatacttcgaagtgaataagaagggaagcctgattattgctgagatcaccttggtattgccttgtacataaccaagatgtttcacagtgcctccttaagtgctcaggaaagcactttcatttaatttaatttaagctaaattctggagattttgctaaacattgacattaatgcttcatggcttttaagacaaactcatattgctaaaactatttggcagcagtaaatttatgggcagagttattgctcttacatctactgcagtacaaaactcagatgatcagcccttcgattgctcatacttattaaaataaataaataaacatgaaacatcagccacattaaggagtcagggaaactcctgaggaataacaatgtctctggagatgttttcaaatgctaacctgagactcacactgtggtttgggggtttcattattattattattattttatttcagaagaggaaagtaatattatttctcaaaataaaactttggcagagtatgaatcagggaagcagcccacacatggaaaacacaatccacaatctgaaagtagtctaggcaggctcatttttttgttgaaggaattcacatggaggcaattctgctcagttccagagagagattcttatcatcaaaagcacacacaataaccttgcttcaccacctgccactttctccagtggcctcttgttgtgaccagtaattgagaaatgacaaatgggtatagagccaaatctctaaaacagggacaccagtgtctcctagtatctgggtaataacctcctttcagtcttagtccacaccacacactaccctccagtctctcctactctttactgtcacagaaaagactctcagcttttattcacacctgccttcagaaggccaaaccattttgtgcctgaaaactgttacccactcgccccacactttacataagtatcacatatgttctttctacaaattggtatacaggtgccatttaatccattcaaatttggaagctacatcttcaagggtctgagagagctcactccccccatatattccccctttacatgttttcttataagacatacagtttaatcaattaacaaactaaacagcttatatactggcaatatattacagatgggtttatgtcagagtaatagatcacatgaaatggaccatgtggtaccccagtgcattatgtcttggtagagccctgaggacactgacagtagcatctctaagtaagtagtgctgtatgaatacagacacatgcggatctgtatctacatccatctgactaggccaaggagcaggtagatgcaagatagagacacacacatgctggatggggccactgcacaccttgtcatgccatttaaaagggcagttacaggttgccggttttgcagccattaaaattacactttatggaaaaggcttctctaattgtgtctgatttgctttctgtagtaagcatcattggaagaagaccaaagcaagagcaactagaagttaaatatacatttgagcttagctgcaatacagaaccctggggaagaagcaggctgaaagatttatttaattttaggcttggattctctcccttgctgttttcttgatgttgtgtgtctgcatttgtgtgtgtgtgtgtgtctgcgtgtgtgtgtgttccatcacatcatctcctgaagaacgctgggtttcgcaggcaggcggctagtcacctgcaacaacccaggggtcctgccgaggcttccaggctgctgtcagtgtcagatgccagggtctggtcggtggacatggaggagatgtcattgacagacgaggatggagggagactctcactgctgttcactgctgcacctgaaggagaaggctgtccttttactacaccatttttagtcttttcttctgaattcattacttccttgtagataagttctttccattcttcaattgtgtgttctctttcatccaactgcttgtcatatatctgaggtggaggcgcctccacttcggctgggtcataccagacgttgatgtagggatgctgtaaggcgtcgtccactgatattctttttgctgggtcaatcactagcatctttgacaacaagtccctggcttggctggctttgagtttattgtgctcggagtccgctgggaagagggaatctgggaagagtttggggaaggtgagtcccgcatacttgggccgattctccacatagtttcttactgtgggttgcaatttcttcatgaattctggacatggtgttcctagttgttcaattaccttattccactggtcaatatgatcagtgccaggaaacagcactgcaccttttatcatttctcccatgatgcaccctactgaccacatgtcaacgttctccttgtagcccatccccaggatgacctcaggggctctgtaataacgtgtcaccacatatggagtcatcatgaagcttgtgcctgctgtcctggccagtccaaagtccaggattttcaatgtgcaatcagacttgactacaatgttacttggttttaaatccctgtgaataattccagcagaatggaggtgcttaatgccacacaacatttggtacagcaggtaagacattcgctcatggtctaattccatctgaatcacttgacataagttggcatccatcagttccattactaagtaagtttttatggttcacacacttcatgaggaccagctcccggtacgctctcttggcatgtgtttggttctgaaagggtctgctgagcttcttaatggccacatttctgtcaaggacagcatcatacgcggcacaaactatgccctgagccccagagccaataggctttagattctggtagcgcttgagaactgtgaaggttgagtctcccacttccacactgtagaactggttgtcaactttgcttttgctcatgttgtaatgtttggcaatatatgacacatccacttgtttatcgaatccctgacaaaaggcaattttcacatccaatgttggttcactgcagtagtataagaaatggaggctcataaataccacagcttgtatggtttctcatctataggaaacgggtctaattcaacagtttcttgcataagttgccatagtgaagatctgagatgggcctgctgttggtgtttctcacactagccttgggaagaagcatagtcaaataaaaatggaaaccttagtctcagttccactgtgactatgactacccatcagatgttgggcagatagtggctctgtcgacatgtttcttcatctacaatgtatcaggtctagatcacatgataattatggttcttttaccgtgacttcatttatctgggcaatctccacaaatctagaaagtagctttgatgttttcatcagacattattcatttataaactttagagtgccatctgtgtgcc

SEQ ID NO: 9206 - RNA, 4396 nt, Homo sapiens
  source 1..4396: mol_type = other RNA
agacagtagttcttgcctggtttactctgagggggaaattcaccacttatgcaggtacgagagatagcctgtcaagcactttgaagatgctggctggagacttccttctgtcttgtgatgtcatcttgcggctgatgaaattccccttgagactctctttaaagcagcttcctgctctccgcacttaatcccatgtggtataaagtaagggaggggagaagccacagatatatcaagagaaaagtaccgagaaagaaaatcagtaaagaattagagatacagagaggagaagtttttaaaaaaaaaaaaaaaaaacaggaatatgaaagagagggagctcaagtgactgaggaggcatttttaacaatcaggttatctgcaatattaaccagaaaaaaaatggtagcaaaatagagaaaatgggccatttttattccaggggacaagctgcacaaaggaatgttcttctatttattttaaacaaatgactgcgtgtactgaatctgactgtgtgaaataatctcagaatggcagcaccactggcatggcgatggtgcaggtgggtgcagttccctgtggtctctattgcttgaagagagaaagaaagttccctattattatatttaaggcagttttcagagcactggcattcttgtttgctctgttttggggatattctatttgccaatcagttcacactcatcaaccatccacttcctgtctttcacttcttcaggtgaaatatcaccactctagtgagcaccaacatggtcagagtgcaaataactgtgatggatacttcgaagtgaataagaagggaagcctgattattgctgagatcaccttggtattgccttgtacataaccaagatgtttcacagtgcctccttaagtgctcaggaaagcactttcatttaatttaatttaagctaaattctggagattttgctaaacattgacattaatgcttcatggcttttaagacaaactcatattgctaaaactatttggcagcagtaaatttatgggcagagttattgctcttacatctactgcagtacaaaactcagatgatcagcccttcgattgctcatacttattaaaataaataaataaacatgaaacatcagccacattaaggagtcagggaaactcctgaggaataacaatgtctctggagatgttttcaaatgctaacctgagactcacactgtggtttgggggtttcattattattattattattttatttcagaagaggaaagtaatattatttctcaaaataaaactttggcagagtatgaatcagggaagcagcccacacatggaaaacacaatccacaatctgaaagtagtctaggcaggctcatttttttgttgaaggaattcacatggaggcaattctgctcagttccagagagagattcttatcatcaaaagcacacacaataaccttgcttcaccacctgccactttctccagtggcctcttgttgtgaccagtaattgagaaatgacaaatgggtatagagccaaatctctaaaacagggacaccagtgtctcctagtatctgggtaataacctcctttcagtcttagtccacaccacacactaccctccagtctctcctactctttactgtcacagaaaagactctcagcttttattcacacctgccttcagaaggccaaaccattttgtgcctgaaaactgttacccactcgccccacactttacataagtatcacatatgttctttctacaaattggtatacaggtgccatttaatccattcaaatttggaagctacatcttcaagggtctgagagagctcactccccccatatattccccctttacatgttttcttataagacatacagtttaatcaattaacaaactaaacagcttatatactggcaatatattacagatgggtttatgtcagagtaatagatcacatgaaatggaccatgtggtaccccagtgcattatgtcttggtagagccctgaggacactgacagtagcatctctaagtaagtagtgctgtatgaatacagacacatgcggatctgtatctacatccatctgactaggccaaggagcaggtagatgcaagatagagacacacacatgctggatggggccactgcacaccttgtcatgccatttaaaagggcagttacaggttgccggttttgcagccattaaaattacactttatggaaaaggcttctctaattgtgtctgatttgctttctgtagtaagcatcattggaagaagaccaaagcaagagcaactagaagttaaatatacatttgagcttagctgcaatacagaaccctggggaagaagcaggctgaaagatttatttaattttaggcttggattctctcccttgctgttttcttgatgttgtgtgtctgcatttgtgtgtgtgtgtgtgtctgcgtgtgtgtgtgttccatcacatcatctcctgaagaacgctgggtttcgcaggcaggcggctagtcacctgcaacaacccaggggtcctgccgaggcttccaggctgctgtcagtgtcagatgccagggtctggtcggtggacatggaggagatgtcattgacagacgaggatggagggagactctcactgctgttcactgctgcacctgaaggagaaggctgtccttttactacaccatttttagtcttttcttctgaattcattacttccttgtagataagttctttccattcttcaattgtgtgttctctttcatccaactgcttgtcatatatctgaggtggaggcgcctccacttcggctgggtcataccagacgttgatgtagggatgctgtaaggcgtcgtccactgatattctttttgctgggtcaatcactagcatctttgacaacaagtccctggcttggctggctttgagtttattgtgctcggagtccgctgggaagagggaatctgggaagagtttggggaaggtgagtcccgcatacttgggccgattctccacatagtttcttactgtgggttgcaatttcttcatgaattctggacatggtgttcctagttgttcaattaccttattccactggtcaatatgatcagtgccaggaaacagcactgcaccttttatcatttctcccatgatgcaccctactgaccacatgtcaacgttctccttgtagcccatccccaggatgacctcaggggctctgtaataacgtgtcaccacatatggagtcatcatgaagcttgtgcctgctgtcctggccagtccaaagtccaggattttcaatgtgcaatcagacttgactacaatgttacttggttttaaatccctgtgaataattccagcagaatggaggtgcttaatgccacacaacatttggtacagcaggtaagacattcgctcatggtctaattccatctgaatcacttgacataagttggcatccatcagttccattactaagtaagtttttatggttcacacacttcatgaggaccagctcccggtacgctctcttggcatgtgtttggttctgaaagggtctgctgagcttcttaatggccacatttctgtcaaggacagcatcatacgcggcacaaactatgccctgagccccagagccaataggctttagattctggtagcgcttgagaactgtgaaggttgagtctcccacttccacactgtagaactggttgtcaactttgcttttgctcatgttgtaatgtttggcaatatatgacacatccacttgtttatcgaatcccttgttttacctgtaaggaacacacacctgacaaaaggcaattttcacatccaatgttggttcactgcagtagtataagaaatggaggctcataaataccacagcttgtatggtttctcatctataggaaacgggtctaattcaacagtttcttgcataagttgccatagtgaagatctgagatgggcctgctgttggtgtttctcacactagccattccgtgcctgagaactacgatcctgatccggcagtgtttgccccagaaatcctccctacttgtttttcattaaccacattccagactaacatggaagagattctttggagatatggagattgtttaaaattaacgatggacaggtgatttccaagaaaacccaatcttaaactcactcaagcccctaggaattgaggggtgaggacaaaaaaggaaatttgtaaaaatgaaaaaagaaaagaaaaaggtaagcatatagcaagcaccacccacccccataaaaataaaaagtgaaggggaggttaaagaaaatagaagaagagtggcttgctgaatcaccctctttcactgcctggaaaccattgtgcagcgtgatgctgcctgtaccattgt

SEQ ID NO: 9207 - RNA, 4132 nt, Homo sapiens
  source 1..4132: mol_type = other RNA
agacagtagttcttgcctggtttactctgagggggaaattcaccacttatgcaggtacgagagatagcctgtcaagcactttgaagatgctggctggagacttccttctgtcttgtgatgtcatcttgcggctgatgaaattccccttgagactctctttaaagcagcttcctgctctccgcacttaatcccatgtggtataaagtaagggaggggagaagccacagatatatcaagagaaaagtaccgagaaagaaaatcagtaaagaattagagatacagagaggagaagtttttaaaaaaaaaaaaaaaaaacaggaatatgaaagagagggagctcaagtgactgaggaggcatttttaacaatcaggttatctgcaatattaaccagaaaaaaaatggtagcaaaatagagaaaatgggccatttttattccaggggacaagctgcacaaaggaatgttcttctatttattttaaacaaatgactgcgtgtactgaatctgactgtgtgaaataatctcagaatggcagcaccactggcatggcgatggtgcaggtgggtgcagttccctgtggtctctattgcttgaagagagaaagaaagttccctattattatatttaaggcagttttcagagcactggcattcttgtttgctctgttttggggatattctatttgccaatcagttcacactcatcaaccatccacttcctgtctttcacttcttcaggtgaaatatcaccactctagtgagcaccaacatggtcagagtgcaaataactgtgatggatacttcgaagtgaataagaagggaagcctgattattgctgagatcaccttggtattgccttgtacataaccaagatgtttcacagtgcctccttaagtgctcaggaaagcactttcatttaatttaatttaagctaaattctggagattttgctaaacattgacattaatgcttcatggcttttaagacaaactcatattgctaaaactatttggcagcagtaaatttatgggcagagttattgctcttacatctactgcagtacaaaactcagatgatcagcccttcgattgctcatacttattaaaataaataaataaacatgaaacatcagccacattaaggagtcagggaaactcctgaggaataacaatgtctctggagatgttttcaaatgctaacctgagactcacactgtggtttgggggtttcattattattattattattttatttcagaagaggaaagtaatattatttctcaaaataaaactttggcagagtatgaatcagggaagcagcccacacatggaaaacacaatccacaatctgaaagtagtctaggcaggctcatttttttgttgaaggaattcacatggaggcaattctgctcagttccagagagagattcttatcatcaaaagcacacacaataaccttgcttcaccacctgccactttctccagtggcctcttgttgtgaccagtaattgagaaatgacaaatgggtatagagccaaatctctaaaacagggacaccagtgtctcctagtatctgggtaataacctcctttcagtcttagtccacaccacacactaccctccagtctctcctactctttactgtcacagaaaagactctcagcttttattcacacctgccttcagaaggccaaaccattttgtgcctgaaaactgttacccactcgccccacactttacataagtatcacatatgttctttctacaaattggtatacaggtgccatttaatccattcaaatttggaagctacatcttcaagggtctgagagagctcactccccccatatattccccctttacatgttttcttataagacatacagtttaatcaattaacaaactaaacagcttatatactggcaatatattacagatgggtttatgtcagagtaatagatcacatgaaatggaccatgtggtaccccagtgcattatgtcttggtagagccctgaggacactgacagtagcatctctaagtaagtagtgctgtatgaatacagacacatgcggatctgtatctacatccatctgactaggccaaggagcaggtagatgcaagatagagacacacacatgctggatggggccactgcacaccttgtcatgccatttaaaagggcagttacaggttgccggttttgcagccattaaaattacactttatggaaaaggcttctctaattgtgtctgatttgctttctgtagtaagcatcattggaagaagaccaaagcaagagcaactagaagttaaatatacatttgagcttagctgcaatacagaaccctggggaagaagcaggctgaaagatttatttaattttaggcttggattctctcccttgctgttttcttgatgttgtgtgtctgcatttgtgtgtgtgtgtgtgtctgcgtgtgtgtgtgttccatcacatcatctcctgaagaacgctgggtttcgcaggcaggcggctagtcacctgcaacaacccaggggtcctgccgaggcttccaggctgctgtcagtgtcagatgccagggtctggtcggtggacatggaggagatgtcattgacagacgaggatggagggagactctcactgctgttcactgctgcacctgtgctgaaggagaaggctgtccttttactacaccatttttagtcttttcttctgaattcattacttccttgtagataagttctttccattcttcaattgtgtgttctctttcatccaactgcttgtcatatatctgaggtggaggcgcctccacttcggctgggtcataccagacgttgatgtagggatgctgtaaggcgtcgtccactgatattctttttgctgggtcaatcactagcatctttgacaacaagtccctggcttggctggctttgagtttattgtgctcggagtccgctgggaagagggaatctgggaagagtttggggaaggtgagtcccgcatacttgggccgattctccacatagtttcttactgtgggttgcaatttcttcatgaattctggacatggtgttcctagttgttcaattaccttattccactggtcaatatagtcccttcctggaaagaggattttgtggcgaaccatttctcccataatgcatcccacagaccatatatccacgttctccttgtagcccatccccaggatgacctcaggggctctgtaataacgtgtcaccacatatggagtcatcatgaagcttgtgcctgctgtcctggccagtccaaagtccaggattttcaatgtgcaatcagacttgactacaatgttacttggttttaaatccctgtgaataattccagcagaatggaggtgcttaatgccacacaacatttggtacagcaggtaagacattcgctcatggtctaattccatctgaatcacttgacataagttggcatccatcagttccattactaagtaaacatcttggaactcctccagcgttttctggggtgtgaagacatttaataaactaataatgtttttatggttcacacacttcatgaggaccagctcccggtacgctctcttggcatgtgtttggttctgaaagggtctgctgagcttcttaatggccacatttctgtcaaggacagcatcatacgcggcacaaactatgccctgagccccagagccaataggctttagattctggtagcgcttgagaactgtgaaggttgagtctcccacttccacactgtagaactggttgtcaactttgcttttgctcatgttgtaatgtttggcaatatatgacacatccacttgtttatcgaatccctgacaaaaggcaattttcacatccaatgttggttcactgcagtagtataagaaatggaggctcataaataccacagcttgtatggtttctcatctataggaaacgggtctaattcaacagtttcttgcataagttgccatagtgaagatctgagatgggcctgctgttggtgtttctcacactagccagacaatgacagcaaaaacacactcagcccctctgggatctgttcataaacatccccttccagcatggcaaacacactcctctcaacagcagat

SEQ ID NO: 9208 - RNA, 4469 nt, Homo sapiens
  source 1..4469: mol_type = other RNA
agacagtagttcttgcctggtttactctgagggggaaattcaccacttatgcaggtacgagagatagcctgtcaagcactttgaagatgctggctggagacttccttctgtcttgtgatgtcatcttgcggctgatgaaattccccttgagactctctttaaagcagcttcctgctctccgcacttaatcccatgtggtataaagtaagggaggggagaagccacagatatatcaagagaaaagtaccgagaaagaaaatcagtaaagaattagagatacagagaggagaagtttttaaaaaaaaaaaaaaaaaacaggaatatgaaagagagggagctcaagtgactgaggaggcatttttaacaatcaggttatctgcaatattaaccagaaaaaaaatggtagcaaaatagagaaaatgggccatttttattccaggggacaagctgcacaaaggaatgttcttctatttattttaaacaaatgactgcgtgtactgaatctgactgtgtgaaataatctcagaatggcagcaccactggcatggcgatggtgcaggtgggtgcagttccctgtggtctctattgcttgaagagagaaagaaagttccctattattatatttaaggcagttttcagagcactggcattcttgtttgctctgttttggggatattctatttgccaatcagttcacactcatcaaccatccacttcctgtctttcacttcttcaggtgaaatatcaccactctagtgagcaccaacatggtcagagtgcaaataactgtgatggatacttcgaagtgaataagaagggaagcctgattattgctgagatcaccttggtattgccttgtacataaccaagatgtttcacagtgcctccttaagtgctcaggaaagcactttcatttaatttaatttaagctaaattctggagattttgctaaacattgacattaatgcttcatggcttttaagacaaactcatattgctaaaactatttggcagcagtaaatttatgggcagagttattgctcttacatctactgcagtacaaaactcagatgatcagcccttcgattgctcatacttattaaaataaataaataaacatgaaacatcagccacattaaggagtcagggaaactcctgaggaataacaatgtctctggagatgttttcaaatgctaacctgagactcacactgtggtttgggggtttcattattattattattattttatttcagaagaggaaagtaatattatttctcaaaataaaactttggcagagtatgaatcagggaagcagcccacacatggaaaacacaatccacaatctgaaagtagtctaggcaggctcatttttttgttgaaggaattcacatggaggcaattctgctcagttccagagagagattcttatcatcaaaagcacacacaataaccttgcttcaccacctgccactttctccagtggcctcttgttgtgaccagtaattgagaaatgacaaatgggtatagagccaaatctctaaaacagggacaccagtgtctcctagtatctgggtaataacctcctttcagtcttagtccacaccacacactaccctccagtctctcctactctttactgtcacagaaaagactctcagcttttattcacacctgccttcagaaggccaaaccattttgtgcctgaaaactgttacccactcgccccacactttacataagtatcacatatgttctttctacaaattggtatacaggtgccatttaatccattcaaatttggaagctacatcttcaagggtctgagagagctcactccccccatatattccccctttacatgttttcttataagacatacagtttaatcaattaacaaactaaacagcttatatactggcaatatattacagatgggtttatgtcagagtaatagatcacatgaaatggaccatgtggtaccccagtgcattatgtcttggtagagccctgaggacactgacagtagcatctctaagtaagtagtgctgtatgaatacagacacatgcggatctgtatctacatccatctgactaggccaaggagcaggtagatgcaagatagagacacacacatgctggatggggccactgcacaccttgtcatgccatttaaaagggcagttacaggttgccggttttgcagccattaaaattacactttatggaaaaggcttctctaattgtgtctgatttgctttctgtagtaagcatcattggaagaagaccaaagcaagagcaactagaagttaaatatacatttgagcttagctgcaatacagaaccctggggaagaagcaggctgaaagatttatttaattttaggcttggattctctcccttgctgttttcttgatgttgtgtgtctgcatttgtgtgtgtgtgtgtgtctgcgtgtgtgtgtgttccatcacatcatctcctgaagaacgctgggtttcgcaggcaggcggctagtcacctgcaacaacccaggggtcctgccgaggcttccaggctgctgtcagtgtcagatgccagggtctggtcggtggacatggaggagatgtcattgacagacgaggatggagggagactctcactgctgttcactgctgcacctgtgctgaaggagaaggctgtccttttactacaccatttttagtcttttcttctgaattcattacttccttgtagataagttctttccattcttcaattgtgtgttctctttcatccaactgcttgtcatatatctgaggtggaggcgcctccacttcggctgggtcataccagacgttgatgtagggatgctgtaaggcgtcgtccactgatattctttttgctgggtcaatcactagcatctttgacaacaagtccctggcttggctggctttgagtttattgtgctcggagtccgctgggaagagggaatctgggaagagtttggggaaggtgagtcccgcatacttgggccgattctccacatagtttcttactgtgggttgcaatttcttcatgaattctggacatggtgttcctagttgttcaattaccttattccactggtcaatatagtcccttcctggaaagaggattttgtggcgaaccatttctcccataatgcatcccacagaccatatatccacgttctccttgtagcccatccccaggatgacctcaggggctctgtaataacgtgtcaccacatatggagtcatcatgaagcttgtgcctgctgtcctggccagtccaaagtccaggattttcaatgtgcaatcagacttgactacaatgttacttggttttaaatccctgtgaataattccagcagaatggaggtgcttaatgccacacaacatttggtacagcaggtaagacattcgctcatggtctaattccatctgaatcacttgacataagttggcatccatcagttccattactaagtaaacatcttggaactcctccagcgttttctggggtgtgaagacatttaataaactaataatgtttttatggttcacacacttcatgaggaccagctcccggtacgctctcttggcatgtgtttggttctgaaagggtctgctgagcttcttaatggccacatttctgtcaaggacagcatcatacgcggcacaaactatgccctgagccccagagccaataggctttagattctggtagcgcttgagaactgtgaaggttgagtctcccacttccacactgtagaactggttgtcaactttgcttttgctcatgttgtaatgtttggcaatatatgacacatccacttgtttatcgaatccctgacaaaaggcaattttcacatccaatgttggttcactgcagtagtataagaaatggaggctcataaataccacagcttgtatggtttctcatctataggaaacgggtctaattcaacagtttcttgcataagttgccatagtgaagatctgagatgggcctgctgttggtgtttctcacactagccagaggcagccaaaccgctacatccaaagcatccagcccctaaaatctaatggttctgaagtggagtcagaagcttgtgatatacttatatatttatttgttatatatttgtaacatatatgctcacctaaagtagaaaattcacagaagcttctctgagagaaatggtccttactgcaactattttaaatatgttgataagcattctgtgttatcttccagggtccgacaactagccgatgagggatagaaggagatattggatgttgtgctggcaatgcctggtgcacttacactcgttttccttccacctgaactgtagtctatcccatatgacttagcctgcttccttgcagtttgttcataaaagttatcatcaacatggccagaagcaggcagggctgctgtacagacactgtcaggctctgcacc

SEQ ID NO: 9209 - RNA, 4440 nt, Homo sapiens
  source 1..4440: mol_type = other RNA
agacagtagttcttgcctggtttactctgagggggaaattcaccacttatgcaggtacgagagatagcctgtcaagcactttgaagatgctggctggagacttccttctgtcttgtgatgtcatcttgcggctgatgaaattccccttgagactctctttaaagcagcttcctgctctccgcacttaatcccatgtggtataaagtaagggaggggagaagccacagatatatcaagagaaaagtaccgagaaagaaaatcagtaaagaattagagatacagagaggagaagtttttaaaaaaaaaaaaaaaaaacaggaatatgaaagagagggagctcaagtgactgaggaggcatttttaacaatcaggttatctgcaatattaaccagaaaaaaaatggtagcaaaatagagaaaatgggccatttttattccaggggacaagctgcacaaaggaatgttcttctatttattttaaacaaatgactgcgtgtactgaatctgactgtgtgaaataatctcagaatggcagcaccactggcatggcgatggtgcaggtgggtgcagttccctgtggtctctattgcttgaagagagaaagaaagttccctattattatatttaaggcagttttcagagcactggcattcttgtttgctctgttttggggatattctatttgccaatcagttcacactcatcaaccatccacttcctgtctttcacttcttcaggtgaaatatcaccactctagtgagcaccaacatggtcagagtgcaaataactgtgatggatacttcgaagtgaataagaagggaagcctgattattgctgagatcaccttggtattgccttgtacataaccaagatgtttcacagtgcctccttaagtgctcaggaaagcactttcatttaatttaatttaagctaaattctggagattttgctaaacattgacattaatgcttcatggcttttaagacaaactcatattgctaaaactatttggcagcagtaaatttatgggcagagttattgctcttacatctactgcagtacaaaactcagatgatcagcccttcgattgctcatacttattaaaataaataaataaacatgaaacatcagccacattaaggagtcagggaaactcctgaggaataacaatgtctctggagatgttttcaaatgctaacctgagactcacactgtggtttgggggtttcattattattattattattttatttcagaagaggaaagtaatattatttctcaaaataaaactttggcagagtatgaatcagggaagcagcccacacatggaaaacacaatccacaatctgaaagtagtctaggcaggctcatttttttgttgaaggaattcacatggaggcaattctgctcagttccagagagagattcttatcatcaaaagcacacacaataaccttgcttcaccacctgccactttctccagtggcctcttgttgtgaccagtaattgagaaatgacaaatgggtatagagccaaatctctaaaacagggacaccagtgtctcctagtatctgggtaataacctcctttcagtcttagtccacaccacacactaccctccagtctctcctactctttactgtcacagaaaagactctcagcttttattcacacctgccttcagaaggccaaaccattttgtgcctgaaaactgttacccactcgccccacactttacataagtatcacatatgttctttctacaaattggtatacaggtgccatttaatccattcaaatttggaagctacatcttcaagggtctgagagagctcactccccccatatattccccctttacatgttttcttataagacatacagtttaatcaattaacaaactaaacagcttatatactggcaatatattacagatgggtttatgtcagagtaatagatcacatgaaatggaccatgtggtaccccagtgcattatgtcttggtagagccctgaggacactgacagtagcatctctaagtaagtagtgctgtatgaatacagacacatgcggatctgtatctacatccatctgactaggccaaggagcaggtagatgcaagatagagacacacacatgctggatggggccactgcacaccttgtcatgccatttaaaagggcagttacaggttgccggttttgcagccattaaaattacactttatggaaaaggcttctctaattgtgtctgatttgctttctgtagtaagcatcattggaagaagaccaaagcaagagcaactagaagttaaatatacatttgagcttagctgcaatacagaaccctggggaagaagcaggctgaaagatttatttaattttaggcttggattctctcccttgctgttttcttgatgttgtgtgtctgcatttgtgtgtgtgtgtgtgtctgcgtgtgtgtgtgttccatcacatcatctcctgaagaacgctgggtttcgcaggcaggcggctagtcacctgcaacaacccaggggtcctgccgaggcttccaggctgctgtcagtgtcagatgccagggtctggtcggtggacatggaggagatgtcattgacagacgaggatggagggagactctcactgctgttcactgctgcacctgtgctgaaggagaaggctgtccttttactacaccatttttagtcttttcttctgaattcattacttccttgtagataagttctttccattcttcaattgtgtgttctctttcatccaactgcttgtcatatatctgaggtggaggcgcctccacttcggctgggtcataccagacgttgatgtagggatgctgtaaggcgtcgtccactgatattctttttgctgggtcaatcactagcatctttgacaacaagtccctggcttggctggctttgagtttattgtgctcggagtccgctgggaagagggaatctgggaagagtttggggaaggtgagtcccgcatacttgggccgattctccacatagtttcttactgtgggttgcaatttcttcatgaattctggacatggtgttcctagttgttcaattaccttattccactggtcaatatagtcccttcctggaaagaggattttgtggcgaaccatttctcccataatgcatcccacagaccatatatccacgttctccttgtagcccatccccaggatgacctcaggggctctgtaataacgtgtcaccacatatggagtcatcatgaagcttgtgcctgctgtcctggccagtccaaagtccaggattttcaatgtgcaatcagacttgactacaatgttacttggttttaaatccctgtgaataattccagcagaatggaggtgcttaatgccacacaacatttggtacagcaggtaagacattcgctcatggtctaattccatctgaatcacttgacataagttggcatccatcagttccattactaagtaaacatcttggaactcctccagcgttttctggggtgtgaagacatttaataaactaataatgtttttatggttcacacacttcatgaggaccagctcccggtacgctctcttggcatgtgtttggttctgaaagggtctgctgagcttcttaatggccacatttctgtcaaggacagcatcatacgcggcacaaactatgccctgagccccagagccaataggctttagattctggtagcgcttgagaactgtgaaggttgagtctcccacttccacactgtagaactggttgtcaactttgcttttgctcatgttgtaatgtttggcaatatatgacacatccacttgtttatcgaatccctgacaaaaggcaattttcacatccaatgttggttcactgcagtagtataagaaatggaggctcataaataccacagcttgtatggtttctcatctataggaaacgggtctaattcaacagtttcttgcataagttgccatagtgaagatctgagatgggcctgctgttggtgtttctcacactagccattccgtgcctgagaactacgatcctgatccggcagtgtttgccccagaaatcctccctacttgtttttcattaaccacattccagactaacatggaagagattctttggagatatggagattgtttaaaattaacgatggacaggtgatttccaagaaaacccaatcttaaactcactcaagcccctaggaattgaggggtgaggacaaaaaaggaaatttgtaaaaatgaaaaaagaaaagaaaaaggtaagcatatagcaagcaccacccacccccataaaaataaaaagtgaaggggaggttaaagaaaatagaagaagagtggcttgctgaatcaccctctttcactgcctggaaaccattgtgcagcgtgatgctgcctgtaccattgtggaacct

SEQ ID NO: 9210 - RNA, 4204 nt, Homo sapiens
  source 1..4204: mol_type = other RNA
agacagtagttcttgcctggtttactctgagggggaaattcaccacttatgcaggtacgagagatagcctgtcaagcactttgaagatgctggctggagacttccttctgtcttgtgatgtcatcttgcggctgatgaaattccccttgagactctctttaaagcagcttcctgctctccgcacttaatcccatgtggtataaagtaagggaggggagaagccacagatatatcaagagaaaagtaccgagaaagaaaatcagtaaagaattagagatacagagaggagaagtttttaaaaaaaaaaaaaaaaaacaggaatatgaaagagagggagctcaagtgactgaggaggcatttttaacaatcaggttatctgcaatattaaccagaaaaaaaatggtagcaaaatagagaaaatgggccatttttattccaggggacaagctgcacaaaggaatgttcttctatttattttaaacaaatgactgcgtgtactgaatctgactgtgtgaaataatctcagaatggcagcaccactggcatggcgatggtgcaggtgggtgcagttccctgtggtctctattgcttgaagagagaaagaaagttccctattattatatttaaggcagttttcagagcactggcattcttgtttgctctgttttggggatattctatttgccaatcagttcacactcatcaaccatccacttcctgtctttcacttcttcaggtgaaatatcaccactctagtgagcaccaacatggtcagagtgcaaataactgtgatggatacttcgaagtgaataagaagggaagcctgattattgctgagatcaccttggtattgccttgtacataaccaagatgtttcacagtgcctccttaagtgctcaggaaagcactttcatttaatttaatttaagctaaattctggagattttgctaaacattgacattaatgcttcatggcttttaagacaaactcatattgctaaaactatttggcagcagtaaatttatgggcagagttattgctcttacatctactgcagtacaaaactcagatgatcagcccttcgattgctcatacttattaaaataaataaataaacatgaaacatcagccacattaaggagtcagggaaactcctgaggaataacaatgtctctggagatgttttcaaatgctaacctgagactcacactgtggtttgggggtttcattattattattattattttatttcagaagaggaaagtaatattatttctcaaaataaaactttggcagagtatgaatcagggaagcagcccacacatggaaaacacaatccacaatctgaaagtagtctaggcaggctcatttttttgttgaaggaattcacatggaggcaattctgctcagttccagagagagattcttatcatcaaaagcacacacaataaccttgcttcaccacctgccactttctccagtggcctcttgttgtgaccagtaattgagaaatgacaaatgggtatagagccaaatctctaaaacagggacaccagtgtctcctagtatctgggtaataacctcctttcagtcttagtccacaccacacactaccctccagtctctcctactctttactgtcacagaaaagactctcagcttttattcacacctgccttcagaaggccaaaccattttgtgcctgaaaactgttacccactcgccccacactttacataagtatcacatatgttctttctacaaattggtatacaggtgccatttaatccattcaaatttggaagctacatcttcaagggtctgagagagctcactccccccatatattccccctttacatgttttcttataagacatacagtttaatcaattaacaaactaaacagcttatatactggcaatatattacagatgggtttatgtcagagtaatagatcacatgaaatggaccatgtggtaccccagtgcattatgtcttggtagagccctgaggacactgacagtagcatctctaagtaagtagtgctgtatgaatacagacacatgcggatctgtatctacatccatctgactaggccaaggagcaggtagatgcaagatagagacacacacatgctggatggggccactgcacaccttgtcatgccatttaaaagggcagttacaggttgccggttttgcagccattaaaattacactttatggaaaaggcttctctaattgtgtctgatttgctttctgtagtaagcatcattggaagaagaccaaagcaagagcaactagaagttaaatatacatttgagcttagctgcaatacagaaccctggggaagaagcaggctgaaagatttatttaattttaggcttggattctctcccttgctgttttcttgatgttgtgtgtctgcatttgtgtgtgtgtgtgtgtctgcgtgtgtgtgtgttccatcacatcatctcctgaagaacgctgggtttcgcaggcaggcggctagtcacctgcaacaacccaggggtcctgccgaggcttccaggctgctgtcagtgtcagatgccagggtctggtcggtggacatggaggagatgtcattgacagacgaggatggagggagactctcactgctgttcactgctgcacctgtgctgaaggagaaggctgtccttttactacaccatttttagtcttttcttctgaattcattacttccttgtagataagttctttccattcttcaattgtgtgttctctttcatccaactgcttgtcatatatctgaggtggaggcgcctccacttcggctgggtcataccagacgttgatgtagggatgctgtaaggcgtcgtccactgatattctttttgctgggtcaatcactagcatctttgacaacaagtccctggcttggctggctttgagtttattgtgctcggagtccgctgggaagagggaatctgggaagagtttggggaaggtgagtcccgcatacttgggccgattctccacatagtttcttactgtgggttgcaatttcttcatgaattctggacatggtgttcctagttgttcaattaccttattccactggtcaatatagtcccttcctggaaagaggattttgtggcgaaccatttctcccataatgcatcccacagaccatatatccacgttctccttgtagcccatccccaggatgacctcaggggctctgtaataacgtgtcaccacatatggagtcatcatgaagcttgtgcctgctgtcctggccagtccaaagtccaggattttcaatgtgcaatcagacttgactacaatgttacttggttttaaatccctgtgaataattccagcagaatggaggtgcttaatgccacacaacatttggtacagcaggtaagacattcgctcatggtctaattccatctgaatcacttgacataagttggcatccatcagttccattactaagtaaacatcttggaactcctccagcgttttctggggtgtgaagacatttaataaactaataatgtttttatggttcacacacttcatgaggaccagctcccggtacgctctcttggcatgtgtttggttctgaaagggtctgctgagcttcttaatggccacatttctgtcaaggacagcatcatacgcggcacaaactatgccctgagccccagagccaataggctttagattctggtagcgcttgagaactgtgaaggttgagtctcccacttccacactgtagaactggttgtcaactttgcttttgctcatgttgtaatgtttggcaatatatgacacatccacttgtttatcgaatccctgacaaaaggcaattttcacatccaatgttggttcactgcagtagtataagaaatggaggctcataaataccacagcttgtatggtttctcatctataggaaacgggtctaattcaacagtttcttgcataagttgccatagtgaagatctgagatgggcctgctgttggtgtttctcacactagcctaaagtagaaaattcacagaagcttctctgagagaaatggtccttactgcaactattttaaatatgttgataagcattctgtgttatcttccagggtccgacaactagccgatgagggatagaaggagatattggatgttgtgctggcaatgcctggtgcacttac

SEQ ID NO: 9211 - RNA, 4198 nt, Homo sapiens
  source 1..4198: mol_type = other RNA
agacagtagttcttgcctggtttactctgagggggaaattcaccacttatgcaggtacgagagatagcctgtcaagcactttgaagatgctggctggagacttccttctgtcttgtgatgtcatcttgcggctgatgaaattccccttgagactctctttaaagcagcttcctgctctccgcacttaatcccatgtggtataaagtaagggaggggagaagccacagatatatcaagagaaaagtaccgagaaagaaaatcagtaaagaattagagatacagagaggagaagtttttaaaaaaaaaaaaaaaaaacaggaatatgaaagagagggagctcaagtgactgaggaggcatttttaacaatcaggttatctgcaatattaaccagaaaaaaaatggtagcaaaatagagaaaatgggccatttttattccaggggacaagctgcacaaaggaatgttcttctatttattttaaacaaatgactgcgtgtactgaatctgactgtgtgaaataatctcagaatggcagcaccactggcatggcgatggtgcaggtgggtgcagttccctgtggtctctattgcttgaagagagaaagaaagttccctattattatatttaaggcagttttcagagcactggcattcttgtttgctctgttttggggatattctatttgccaatcagttcacactcatcaaccatccacttcctgtctttcacttcttcaggtgaaatatcaccactctagtgagcaccaacatggtcagagtgcaaataactgtgatggatacttcgaagtgaataagaagggaagcctgattattgctgagatcaccttggtattgccttgtacataaccaagatgtttcacagtgcctccttaagtgctcaggaaagcactttcatttaatttaatttaagctaaattctggagattttgctaaacattgacattaatgcttcatggcttttaagacaaactcatattgctaaaactatttggcagcagtaaatttatgggcagagttattgctcttacatctactgcagtacaaaactcagatgatcagcccttcgattgctcatacttattaaaataaataaataaacatgaaacatcagccacattaaggagtcagggaaactcctgaggaataacaatgtctctggagatgttttcaaatgctaacctgagactcacactgtggtttgggggtttcattattattattattattttatttcagaagaggaaagtaatattatttctcaaaataaaactttggcagagtatgaatcagggaagcagcccacacatggaaaacacaatccacaatctgaaagtagtctaggcaggctcatttttttgttgaaggaattcacatggaggcaattctgctcagttccagagagagattcttatcatcaaaagcacacacaataaccttgcttcaccacctgccactttctccagtggcctcttgttgtgaccagtaattgagaaatgacaaatgggtatagagccaaatctctaaaacagggacaccagtgtctcctagtatctgggtaataacctcctttcagtcttagtccacaccacacactaccctccagtctctcctactctttactgtcacagaaaagactctcagcttttattcacacctgccttcagaaggccaaaccattttgtgcctgaaaactgttacccactcgccccacactttacataagtatcacatatgttctttctacaaattggtatacaggtgccatttaatccattcaaatttggaagctacatcttcaagggtctgagagagctcactccccccatatattccccctttacatgttttcttataagacatacagtttaatcaattaacaaactaaacagcttatatactggcaatatattacagatgggtttatgtcagagtaatagatcacatgaaatggaccatgtggtaccccagtgcattatgtcttggtagagccctgaggacactgacagtagcatctctaagtaagtagtgctgtatgaatacagacacatgcggatctgtatctacatccatctgactaggccaaggagcaggtagatgcaagatagagacacacacatgctggatggggccactgcacaccttgtcatgccatttaaaagggcagttacaggttgccggttttgcagccattaaaattacactttatggaaaaggcttctctaattgtgtctgatttgctttctgtagtaagcatcattggaagaagaccaaagcaagagcaactagaagttaaatatacatttgagcttagctgcaatacagaaccctggggaagaagcaggctgaaagatttatttaattttaggcttggattctctcccttgctgttttcttgatgttgtgtgtctgcatttgtgtgtgtgtgtgtgtctgcgtgtgtgtgtgttccatcacatcatctcctgaagaacgctgggtttcgcaggcaggcggctagtcacctgcaacaacccaggggtcctgccgaggcttccaggctgctgtcagtgtcagatgccagggtctggtcggtggacatggaggagatgtcattgacagacgaggatggagggagactctcactgctgttcactgctgcacctgtgctgaaggagaaggctgtccttttactacaccatttttagtcttttcttctgaattcattacttccttgtagataagttctttccattcttcaattgtgtgttctctttcatccaactgcttgtcatatatctgaggtggaggcgcctccacttcggctgggtcataccagacgttgatgtagggatgctgtaaggcgtcgtccactgatattctttttgctgggtcaatcactagcatctttgacaacaagtccctggcttggctggctttgagtttattgtgctcggagtccgctgggaagagggaatctgggaagagtttggggaaggtgagtcccgcatacttgggccgattctccacatagtttcttactgtgggttgcaatttcttcatgaattctggacatggtgttcctagttgttcaattaccttattccactggtcaatatagtcccttcctggaaagaggattttgtggcgaaccatttctcccataatgcatcccacagaccatatatccacgttctccttgtagcccatccccaggatgacctcaggggctctgtaataacgtgtcaccacatatggagtcatcatgaagcttgtgcctgctgtcctggccagtccaaagtccaggattttcaatgtgcaatcagacttgactacaatgttacttggttttaaatccctgtgaataattccagcagaatggaggtgcttaatgccacacaacatttggtacagcaggtaagacattcgctcatggtctaattccatctgaatcacttgacataagttggcatccatcagttccattactaagtaaacatcttggaactcctccagcgttttctggggtgtgaagacatttaataaactaataatgtttttatggttcacacacttcatgaggaccagctcccggtacgctctcttggcatgtgtttggttctgaaagggtctgctgagcttcttaatggccacatttctgtcaaggacagcatcatacgcggcacaaactatgccctgagccccagagccaataggctttagattctggtagcgcttgagaactgtgaaggttgagtctcccacttccacactgtagaactggttgtcaactttgcttttgctcatgttgtaatgtttggcaatatatgacacatccacttgtttatcgaatccctgacaaaaggcaattttcacatccaatgttggttcactgcagtagtataagaaatggaggctcataaataccacagcttgtatggtttctcatctataggaaacgggtctaattcaacagtttcttgcataagttgccatagtgaagatctgagatgggcctgctgttggtgtttctcacactagcctgatgtctcctcttaagagtttctaccaagattcacaataagaaatacagcttctccctattaaatacagaaaacaaaagatatgcaaaacacaggttttgtattttccccttctttgccttgatcggttcatgaggataaaatgtactcaaactgaaaa

SEQ ID NO: 9212 - RNA, 4203 nt, Homo sapiens
  source 1..4203: mol_type = other RNA
agacagtagttcttgcctggtttactctgagggggaaattcaccacttatgcaggtacgagagatagcctgtcaagcactttgaagatgctggctggagacttccttctgtcttgtgatgtcatcttgcggctgatgaaattccccttgagactctctttaaagcagcttcctgctctccgcacttaatcccatgtggtataaagtaagggaggggagaagccacagatatatcaagagaaaagtaccgagaaagaaaatcagtaaagaattagagatacagagaggagaagtttttaaaaaaaaaaaaaaaaaacaggaatatgaaagagagggagctcaagtgactgaggaggcatttttaacaatcaggttatctgcaatattaaccagaaaaaaaatggtagcaaaatagagaaaatgggccatttttattccaggggacaagctgcacaaaggaatgttcttctatttattttaaacaaatgactgcgtgtactgaatctgactgtgtgaaataatctcagaatggcagcaccactggcatggcgatggtgcaggtgggtgcagttccctgtggtctctattgcttgaagagagaaagaaagttccctattattatatttaaggcagttttcagagcactggcattcttgtttgctctgttttggggatattctatttgccaatcagttcacactcatcaaccatccacttcctgtctttcacttcttcaggtgaaatatcaccactctagtgagcaccaacatggtcagagtgcaaataactgtgatggatacttcgaagtgaataagaagggaagcctgattattgctgagatcaccttggtattgccttgtacataaccaagatgtttcacagtgcctccttaagtgctcaggaaagcactttcatttaatttaatttaagctaaattctggagattttgctaaacattgacattaatgcttcatggcttttaagacaaactcatattgctaaaactatttggcagcagtaaatttatgggcagagttattgctcttacatctactgcagtacaaaactcagatgatcagcccttcgattgctcatacttattaaaataaataaataaacatgaaacatcagccacattaaggagtcagggaaactcctgaggaataacaatgtctctggagatgttttcaaatgctaacctgagactcacactgtggtttgggggtttcattattattattattattttatttcagaagaggaaagtaatattatttctcaaaataaaactttggcagagtatgaatcagggaagcagcccacacatggaaaacacaatccacaatctgaaagtagtctaggcaggctcatttttttgttgaaggaattcacatggaggcaattctgctcagttccagagagagattcttatcatcaaaagcacacacaataaccttgcttcaccacctgccactttctccagtggcctcttgttgtgaccagtaattgagaaatgacaaatgggtatagagccaaatctctaaaacagggacaccagtgtctcctagtatctgggtaataacctcctttcagtcttagtccacaccacacactaccctccagtctctcctactctttactgtcacagaaaagactctcagcttttattcacacctgccttcagaaggccaaaccattttgtgcctgaaaactgttacccactcgccccacactttacataagtatcacatatgttctttctacaaattggtatacaggtgccatttaatccattcaaatttggaagctacatcttcaagggtctgagagagctcactccccccatatattccccctttacatgttttcttataagacatacagtttaatcaattaacaaactaaacagcttatatactggcaatatattacagatgggtttatgtcagagtaatagatcacatgaaatggaccatgtggtaccccagtgcattatgtcttggtagagccctgaggacactgacagtagcatctctaagtaagtagtgctgtatgaatacagacacatgcggatctgtatctacatccatctgactaggccaaggagcaggtagatgcaagatagagacacacacatgctggatggggccactgcacaccttgtcatgccatttaaaagggcagttacaggttgccggttttgcagccattaaaattacactttatggaaaaggcttctctaattgtgtctgatttgctttctgtagtaagcatcattggaagaagaccaaagcaagagcaactagaagttaaatatacatttgagcttagctgcaatacagaaccctggggaagaagcaggctgaaagatttatttaattttaggcttggattctctcccttgctgttttcttgatgttgtgtgtctgcatttgtgtgtgtgtgtgtgtctgcgtgtgtgtgtgttccatcacatcatctcctgaagaacgctgggtttcgcaggcaggcggctagtcacctgcaacaacccaggggtcctgccgaggcttccaggctgctgtcagtgtcagatgccagggtctggtcggtggacatggaggagatgtcattgacagacgaggatggagggagactctcactgctgttcactgctgcacctgtgctgaaggagaaggctgtccttttactacaccatttttagtcttttcttctgaattcattacttccttgtagataagttctttccattcttcaattgtgtgttctctttcatccaactgcttgtcatatatctgaggtggaggcgcctccacttcggctgggtcataccagacgttgatgtagggatgctgtaaggcgtcgtccactgatattctttttgctgggtcaatcactagcatctttgacaacaagtccctggcttggctggctttgagtttattgtgctcggagtccgctgggaagagggaatctgggaagagtttggggaaggtgagtcccgcatacttgggccgattctccacatagtttcttactgtgggttgcaatttcttcatgaattctggacatggtgttcctagttgttcaattaccttattccactggtcaatatagtcccttcctggaaagaggattttgtggcgaaccatttctcccataatgcatcccacagaccatatatccacgttctccttgtagcccatccccaggatgacctcaggggctctgtaataacgtgtcaccacatatggagtcatcatgaagcttgtgcctgctgtcctggccagtccaaagtccaggattttcaatgtgcaatcagacttgactacaatgttacttggttttaaatccctgtgaataattccagcagaatggaggtgcttaatgccacacaacatttggtacagcaggtaagacattcgctcatggtctaattccatctgaatcacttgacataagttggcatccatcagttccattactaagtaaacatcttggaactcctccagcgttttctggggtgtgaagacatttaataaactaataatgtttttatggttcacacacttcatgaggaccagctcccggtacgctctcttggcatgtgtttggttctgaaagggtctgctgagcttcttaatggccacatttctgtcaaggacagcatcatacgcggcacaaactatgccctgagccccagagccaataggctttagattctggtagcgcttgagaactgtgaaggttgagtctcccacttccacactgtagaactggttgtcaactttgcttttgctcatgttgtaatgtttggcaatatatgacacatccacttgtttatcgaatccctgacaaaaggcaattttcacatccaatgttggttcactgcagtagtataagaaatggaggctcataaataccacagcttgtatggtttctcatctataggaaacgggtctaattcaacagtttcttgcataagttgccatagtgaagatctgagatgggcctgctgttggtgtttctcacactagcctggagctgagtcaatttagagagctgcgtgaaatacaggggtagaggaagcagcggcaaaatccctctgggctcgctgggtcccctgccacgccatttctgcctggcctcacaggggtccttgaggagggctgctggaggcactgggaaagctgcagggagaagg

SEQ ID NO: 9213 - RNA, 4342 nt, Homo sapiens
  source 1..4342: mol_type = other RNA
agacagtagttcttgcctggtttactctgagggggaaattcaccacttatgcaggtacgagagatagcctgtcaagcactttgaagatgctggctggagacttccttctgtcttgtgatgtcatcttgcggctgatgaaattccccttgagactctctttaaagcagcttcctgctctccgcacttaatcccatgtggtataaagtaagggaggggagaagccacagatatatcaagagaaaagtaccgagaaagaaaatcagtaaagaattagagatacagagaggagaagtttttaaaaaaaaaaaaaaaaaacaggaatatgaaagagagggagctcaagtgactgaggaggcatttttaacaatcaggttatctgcaatattaaccagaaaaaaaatggtagcaaaatagagaaaatgggccatttttattccaggggacaagctgcacaaaggaatgttcttctatttattttaaacaaatgactgcgtgtactgaatctgactgtgtgaaataatctcagaatggcagcaccactggcatggcgatggtgcaggtgggtgcagttccctgtggtctctattgcttgaagagagaaagaaagttccctattattatatttaaggcagttttcagagcactggcattcttgtttgctctgttttggggatattctatttgccaatcagttcacactcatcaaccatccacttcctgtctttcacttcttcaggtgaaatatcaccactctagtgagcaccaacatggtcagagtgcaaataactgtgatggatacttcgaagtgaataagaagggaagcctgattattgctgagatcaccttggtattgccttgtacataaccaagatgtttcacagtgcctccttaagtgctcaggaaagcactttcatttaatttaatttaagctaaattctggagattttgctaaacattgacattaatgcttcatggcttttaagacaaactcatattgctaaaactatttggcagcagtaaatttatgggcagagttattgctcttacatctactgcagtacaaaactcagatgatcagcccttcgattgctcatacttattaaaataaataaataaacatgaaacatcagccacattaaggagtcagggaaactcctgaggaataacaatgtctctggagatgttttcaaatgctaacctgagactcacactgtggtttgggggtttcattattattattattattttatttcagaagaggaaagtaatattatttctcaaaataaaactttggcagagtatgaatcagggaagcagcccacacatggaaaacacaatccacaatctgaaagtagtctaggcaggctcatttttttgttgaaggaattcacatggaggcaattctgctcagttccagagagagattcttatcatcaaaagcacacacaataaccttgcttcaccacctgccactttctccagtggcctcttgttgtgaccagtaattgagaaatgacaaatgggtatagagccaaatctctaaaacagggacaccagtgtctcctagtatctgggtaataacctcctttcagtcttagtccacaccacacactaccctccagtctctcctactctttactgtcacagaaaagactctcagcttttattcacacctgccttcagaaggccaaaccattttgtgcctgaaaactgttacccactcgccccacactttacataagtatcacatatgttctttctacaaattggtatacaggtgccatttaatccattcaaatttggaagctacatcttcaagggtctgagagagctcactccccccatatattccccctttacatgttttcttataagacatacagtttaatcaattaacaaactaaacagcttatatactggcaatatattacagatgggtttatgtcagagtaatagatcacatgaaatggaccatgtggtaccccagtgcattatgtcttggtagagccctgaggacactgacagtagcatctctaagtaagtagtgctgtatgaatacagacacatgcggatctgtatctacatccatctgactaggccaaggagcaggtagatgcaagatagagacacacacatgctggatggggccactgcacaccttgtcatgccatttaaaagggcagttacaggttgccggttttgcagccattaaaattacactttatggaaaaggcttctctaattgtgtctgatttgctttctgtagtaagcatcattggaagaagaccaaagcaagagcaactagaagttaaatatacatttgagcttagctgcaatacagaaccctggggaagaagcaggctgaaagatttatttaattttaggcttggattctctcccttgctgttttcttgatgttgtgtgtctgcatttgtgtgtgtgtgtgtgtctgcgtgtgtgtgtgttccatcacatcatctcctgaagaacgctgggtttcgcaggcaggcggctagtcacctgcaacaacccaggggtcctgccgaggcttccaggctgctgtcagtgtcagatgccagggtctggtcggtggacatggaggagatgtcattgacagacgaggatggagggagactctcactgctgttcactgctgcacctgtgctgaaggagaaggctgtccttttactacaccatttttagtcttttcttctgaattcattacttccttgtagataagttctttccattcttcaattgtgtgttctctttcatccaactgcttgtcatatatctgaggtggaggcgcctccacttcggctgggtcataccagacgttgatgtagggatgctgtaaggcgtcgtccactgatattctttttgctgggtcaatcactagcatctttgacaacaagtccctggcttggctggctttgagtttattgtgctcggagtccgctgggaagagggaatctgggaagagtttggggaaggtgagtcccgcatacttgggccgattctccacatagtttcttactgtgggttgcaatttcttcatgaattctggacatggtgttcctagttgttcaattaccttattccactggtcaatatagtcccttcctggaaagaggattttgtggcgaaccatttctcccataatgcatcccacagaccatatatccacgttctccttgtagcccatccccaggatgacctcaggggctctgtaataacgtgtcaccacatatggagtcatcatgaagcttgtgcctgctgtcctggccagtccaaagtccaggattttcaatgtgcaatcagacttgactacaatgttacttggttttaaatccctgtgaataattccagcagaatggaggtgcttaatgccacacaacatttggtacagcaggtaagacattcgctcatggtctaattccatctgaatcacttgacataagttggcatccatcagttccattactaagtaaacatcttggaactcctccagcgttttctggggtgtgaagacatttaataaactaataatgtttttatggttcacacacttcatgaggaccagctcccggtacgctctcttggcatgtgtttggttctgaaagggtctgctgagcttcttaatggccacatttctgtcaaggacagcatcatacgcggcacaaactatgccctgagccccagagccaataggctttagattctggtagcgcttgagaactgtgaaggttgagtctcccacttccacactgtagaactggttgtcaactttgcttttgctcatgttgtaatgtttggcaatatatgacacatccacttgtttatcgaatccctgacaaaaggcaattttcacatccaatgttggttcactgcagtagtataagaaatggaggctcataaataccacagcttgtatggtttctcatctataggaaacgggtctaattcaacagtttcttgcataagttgccatagtgaagatctgagatgggcctgctgttggtgtttctcacactagcctggagctgagtcaatttagagagctgcgtgaaatacaggggtagaggaagcagcggcaaaatccctctgggctcgctgggtcccctgccacgccatttctgcctggcctcacaggggtccttgaggagggctgctggaggcactgggaaaggcatttttcactctcctcctcactccctagggtcatagttttgattctgaagttagaagtgtgggggtcgtcggctgcattttcaacttggcctaaaagttggagttcaccacactgcaggcgctaggaactctgccgctcggtcaccaacct

SEQ ID NO: 9214 - RNA, 4203 nt, Homo sapiens
  source 1..4203: mol_type = other RNA
agacagtagttcttgcctggtttactctgagggggaaattcaccacttatgcaggtacgagagatagcctgtcaagcactttgaagatgctggctggagacttccttctgtcttgtgatgtcatcttgcggctgatgaaattccccttgagactctctttaaagcagcttcctgctctccgcacttaatcccatgtggtataaagtaagggaggggagaagccacagatatatcaagagaaaagtaccgagaaagaaaatcagtaaagaattagagatacagagaggagaagtttttaaaaaaaaaaaaaaaaaacaggaatatgaaagagagggagctcaagtgactgaggaggcatttttaacaatcaggttatctgcaatattaaccagaaaaaaaatggtagcaaaatagagaaaatgggccatttttattccaggggacaagctgcacaaaggaatgttcttctatttattttaaacaaatgactgcgtgtactgaatctgactgtgtgaaataatctcagaatggcagcaccactggcatggcgatggtgcaggtgggtgcagttccctgtggtctctattgcttgaagagagaaagaaagttccctattattatatttaaggcagttttcagagcactggcattcttgtttgctctgttttggggatattctatttgccaatcagttcacactcatcaaccatccacttcctgtctttcacttcttcaggtgaaatatcaccactctagtgagcaccaacatggtcagagtgcaaataactgtgatggatacttcgaagtgaataagaagggaagcctgattattgctgagatcaccttggtattgccttgtacataaccaagatgtttcacagtgcctccttaagtgctcaggaaagcactttcatttaatttaatttaagctaaattctggagattttgctaaacattgacattaatgcttcatggcttttaagacaaactcatattgctaaaactatttggcagcagtaaatttatgggcagagttattgctcttacatctactgcagtacaaaactcagatgatcagcccttcgattgctcatacttattaaaataaataaataaacatgaaacatcagccacattaaggagtcagggaaactcctgaggaataacaatgtctctggagatgttttcaaatgctaacctgagactcacactgtggtttgggggtttcattattattattattattttatttcagaagaggaaagtaatattatttctcaaaataaaactttggcagagtatgaatcagggaagcagcccacacatggaaaacacaatccacaatctgaaagtagtctaggcaggctcatttttttgttgaaggaattcacatggaggcaattctgctcagttccagagagagattcttatcatcaaaagcacacacaataaccttgcttcaccacctgccactttctccagtggcctcttgttgtgaccagtaattgagaaatgacaaatgggtatagagccaaatctctaaaacagggacaccagtgtctcctagtatctgggtaataacctcctttcagtcttagtccacaccacacactaccctccagtctctcctactctttactgtcacagaaaagactctcagcttttattcacacctgccttcagaaggccaaaccattttgtgcctgaaaactgttacccactcgccccacactttacataagtatcacatatgttctttctacaaattggtatacaggtgccatttaatccattcaaatttggaagctacatcttcaagggtctgagagagctcactccccccatatattccccctttacatgttttcttataagacatacagtttaatcaattaacaaactaaacagcttatatactggcaatatattacagatgggtttatgtcagagtaatagatcacatgaaatggaccatgtggtaccccagtgcattatgtcttggtagagccctgaggacactgacagtagcatctctaagtaagtagtgctgtatgaatacagacacatgcggatctgtatctacatccatctgactaggccaaggagcaggtagatgcaagatagagacacacacatgctggatggggccactgcacaccttgtcatgccatttaaaagggcagttacaggttgccggttttgcagccattaaaattacactttatggaaaaggcttctctaattgtgtctgatttgctttctgtagtaagcatcattggaagaagaccaaagcaagagcaactagaagttaaatatacatttgagcttagctgcaatacagaaccctggggaagaagcaggctgaaagatttatttaattttaggcttggattctctcccttgctgttttcttgatgttgtgtgtctgcatttgtgtgtgtgtgtgtgtctgcgtgtgtgtgtgttccatcacatcatctcctgaagaacgctgggtttcgcaggcaggcggctagtcacctgcaacaacccaggggtcctgccgaggcttccaggctgctgtcagtgtcagatgccagggtctggtcggtggacatggaggagatgtcattgacagacgaggatggagggagactctcactgctgttcactgctgcacctgtgctgaaggagaaggctgtccttttactacaccatttttagtcttttcttctgaattcattacttccttgtagataagttctttccattcttcaattgtgtgttctctttcatccaactgcttgtcatatatctgaggtggaggcgcctccacttcggctgggtcataccagacgttgatgtagggatgctgtaaggcgtcgtccactgatattctttttgctgggtcaatcactagcatctttgacaacaagtccctggcttggctggctttgagtttattgtgctcggagtccgctgggaagagggaatctgggaagagtttggggaaggtgagtcccgcatacttgggccgattctccacatagtttcttactgtgggttgcaatttcttcatgaattctggacatggtgttcctagttgttcaattaccttattccactggtcaatatagtcccttcctggaaagaggattttgtggcgaaccatttctcccataatgcatcccacagaccatatatccacgttctccttgtagcccatccccaggatgacctcaggggctctgtaataacgtgtcaccacatatggagtcatcatgaagcttgtgcctgctgtcctggccagtccaaagtccaggattttcaatgtgcaatcagacttgactacaatgttacttggttttaaatccctgtgaataattccagcagaatggaggtgcttaatgccacacaacatttggtacagcaggtaagacattcgctcatggtctaattccatctgaatcacttgacataagttggcatccatcagttccattactaagtaaacatcttggaactcctccagcgttttctggggtgtgaagacatttaataaactaataatgtttttatggttcacacacttcatgaggaccagctcccggtacgctctcttggcatgtgtttggttctgaaagggtctgctgagcttcttaatggccacatttctgtcaaggacagcatcatacgcggcacaaactatgccctgagccccagagccaataggctttagattctggtagcgcttgagaactgtgaaggttgagtctcccacttccacactgtagaactggttgtcaactttgcttttgctcatgttgtaatgtttggcaatatatgacacatccacttgtttatcgaatccctgacaaaaggcaattttcacatccaatgttggttcactgcagtagtataagaaatggaggctcataaataccacagcttgtatggtttctcatctataggaaacgggtctaattcaacagtttcttgcataagttgccatagtgaagatctgagatgggcctgctgttggtgtttctcacactagcgcatttttcactctcctcctcactccctagggtcatagttttgattctgaagttagaagtgtgggggtcgtcggctgcattttcaacttggcctaaaagttggagttcaccacactgcaggcgctaggaactctgccgctcggtcaccaacctgagcctctggcta

SEQ ID NO: 9215 - RNA, 4100 nt, Homo sapiens
  source 1..4100: mol_type = other RNA
agacagtagttcttgcctggtttactctgagggggaaattcaccacttatgcaggtacgagagatagcctgtcaagcactttgaagatgctggctggagacttccttctgtcttgtgatgtcatcttgcggctgatgaaattccccttgagactctctttaaagcagcttcctgctctccgcacttaatcccatgtggtataaagtaagggaggggagaagccacagatatatcaagagaaaagtaccgagaaagaaaatcagtaaagaattagagatacagagaggagaagtttttaaaaaaaaaaaaaaaaaacaggaatatgaaagagagggagctcaagtgactgaggaggcatttttaacaatcaggttatctgcaatattaaccagaaaaaaaatggtagcaaaatagagaaaatgggccatttttattccaggggacaagctgcacaaaggaatgttcttctatttattttaaacaaatgactgcgtgtactgaatctgactgtgtgaaataatctcagaatggcagcaccactggcatggcgatggtgcaggtgggtgcagttccctgtggtctctattgcttgaagagagaaagaaagttccctattattatatttaaggcagttttcagagcactggcattcttgtttgctctgttttggggatattctatttgccaatcagttcacactcatcaaccatccacttcctgtctttcacttcttcaggtgaaatatcaccactctagtgagcaccaacatggtcagagtgcaaataactgtgatggatacttcgaagtgaataagaagggaagcctgattattgctgagatcaccttggtattgccttgtacataaccaagatgtttcacagtgcctccttaagtgctcaggaaagcactttcatttaatttaatttaagctaaattctggagattttgctaaacattgacattaatgcttcatggcttttaagacaaactcatattgctaaaactatttggcagcagtaaatttatgggcagagttattgctcttacatctactgcagtacaaaactcagatgatcagcccttcgattgctcatacttattaaaataaataaataaacatgaaacatcagccacattaaggagtcagggaaactcctgaggaataacaatgtctctggagatgttttcaaatgctaacctgagactcacactgtggtttgggggtttcattattattattattattttatttcagaagaggaaagtaatattatttctcaaaataaaactttggcagagtatgaatcagggaagcagcccacacatggaaaacacaatccacaatctgaaagtagtctaggcaggctcatttttttgttgaaggaattcacatggaggcaattctgctcagttccagagagagattcttatcatcaaaagcacacacaataaccttgcttcaccacctgccactttctccagtggcctcttgttgtgaccagtaattgagaaatgacaaatgggtatagagccaaatctctaaaacagggacaccagtgtctcctagtatctgggtaataacctcctttcagtcttagtccacaccacacactaccctccagtctctcctactctttactgtcacagaaaagactctcagcttttattcacacctgccttcagaaggccaaaccattttgtgcctgaaaactgttacccactcgccccacactttacataagtatcacatatgttctttctacaaattggtatacaggtgccatttaatccattcaaatttggaagctacatcttcaagggtctgagagagctcactccccccatatattccccctttacatgttttcttataagacatacagtttaatcaattaacaaactaaacagcttatatactggcaatatattacagatgggtttatgtcagagtaatagatcacatgaaatggaccatgtggtaccccagtgcattatgtcttggtagagccctgaggacactgacagtagcatctctaagtaagtagtgctgtatgaatacagacacatgcggatctgtatctacatccatctgactaggccaaggagcaggtagatgcaagatagagacacacacatgctggatggggccactgcacaccttgtcatgccatttaaaagggcagttacaggttgccggttttgcagccattaaaattacactttatggaaaaggcttctctaattgtgtctgatttgctttctgtagtaagcatcattggaagaagaccaaagcaagagcaactagaagttaaatatacatttgagcttagctgcaatacagaaccctggggaagaagcaggctgaaagatttatttaattttaggcttggattctctcccttgctgttttcttgatgttgtgtgtctgcatttgtgtgtgtgtgtgtgtctgcgtgtgtgtgtgttccatcacatcatctcctgaagaacgctgggtttcgcaggcaggcggctagtcacctgcaacaacccaggggtcctgccgaggcttccaggctgctgtcagtgtcagatgccagggtctggtcggtggacatggaggagatgtcattgacagacgaggatggagggagactctcactgctgttcactgctgcacctgtgctgaaggagaaggctgtccttttactacaccatttttagtcttttcttctgaattcattacttccttgtagataagttctttccattcttcaattgtgtgttctctttcatccaactgcttgtcatatatctgaggtggaggcgcctccacttcggctgggtcataccagacgttgatgtagggatgctgtaaggcgtcgtccactgatattctttttgctgggtcaatcactagcatctttgacaacaagtccctggcttggctggctttgagtttattgtgctcggagtccgctgggaagagggaatctgggaagagtttggggaaggtgagtcccgcatacttgggccgattctccacatagtttcttactgtgggttgcaatttcttcatgaattctggacatggtgttcctagttgttcaattaccttattccactggtcaatatagtcccttcctggaaagaggattttgtggcgaaccatttctcccataatgcatcccacagaccatatatccacgttctccttgtagcccatccccaggatgacctcaggggctctgtaataacgtgtcaccacatatggagtcatcatgaagcttgtgcctgctgtcctggccagtccaaagtccaggattttcaatgtgcaatcagacttgactacaatgttacttggttttaaatccctgtgaataattccagcagaatggaggtgcttaatgccacacaacatttggtacagcaggtaagacattcgctcatggtctaattccatctgaatcacttgacataagttggcatccatcagttccattactaagtaaacatcttggaactcctccagcgttttctggggtgtgaagacatttaataaactaataatgtttttatggttcacacacttcatgaggaccagctcccggtacgctctcttggcatgtgtttggttctgaaagggtctgctgagcttcttaatggccacatttctgtcaaggacagcatcatacgcggcacaaactatgccctgagccccagagccaataggctttagattctggtagcgcttgagaactgtgaaggttgagtctcccacttccacactgtagaactggttgtcaactttgcttttgctcatgttgtaatgtttggcaatatatgacacatccacttgtttatcgaatccctgacaaaaggcaattttcacatccaatgttggttcactgcagtagtataagaaatggaggctcataaatacttgtctctgagcctcttctctctcctctccaaccagaaatatgttggatcctgctcataccagctctctagcaccaattgtgaccatcttttttttttttttagacaaagtctggctctgtcgccaggctggagtgcagtggtgcaatcttggctcacagcaacctccgactccctgg

SEQ ID NO: 9216 - RNA, 4450 nt, Homo sapiens
  source 1..4450: mol_type = other RNA
agacagtagttcttgcctggtttactctgagggggaaattcaccacttatgcaggtacgagagatagcctgtcaagcactttgaagatgctggctggagacttccttctgtcttgtgatgtcatcttgcggctgatgaaattccccttgagactctctttaaagcagcttcctgctctccgcacttaatcccatgtggtataaagtaagggaggggagaagccacagatatatcaagagaaaagtaccgagaaagaaaatcagtaaagaattagagatacagagaggagaagtttttaaaaaaaaaaaaaaaaaacaggaatatgaaagagagggagctcaagtgactgaggaggcatttttaacaatcaggttatctgcaatattaaccagaaaaaaaatggtagcaaaatagagaaaatgggccatttttattccaggggacaagctgcacaaaggaatgttcttctatttattttaaacaaatgactgcgtgtactgaatctgactgtgtgaaataatctcagaatggcagcaccactggcatggcgatggtgcaggtgggtgcagttccctgtggtctctattgcttgaagagagaaagaaagttccctattattatatttaaggcagttttcagagcactggcattcttgtttgctctgttttggggatattctatttgccaatcagttcacactcatcaaccatccacttcctgtctttcacttcttcaggtgaaatatcaccactctagtgagcaccaacatggtcagagtgcaaataactgtgatggatacttcgaagtgaataagaagggaagcctgattattgctgagatcaccttggtattgccttgtacataaccaagatgtttcacagtgcctccttaagtgctcaggaaagcactttcatttaatttaatttaagctaaattctggagattttgctaaacattgacattaatgcttcatggcttttaagacaaactcatattgctaaaactatttggcagcagtaaatttatgggcagagttattgctcttacatctactgcagtacaaaactcagatgatcagcccttcgattgctcatacttattaaaataaataaataaacatgaaacatcagccacattaaggagtcagggaaactcctgaggaataacaatgtctctggagatgttttcaaatgctaacctgagactcacactgtggtttgggggtttcattattattattattattttatttcagaagaggaaagtaatattatttctcaaaataaaactttggcagagtatgaatcagggaagcagcccacacatggaaaacacaatccacaatctgaaagtagtctaggcaggctcatttttttgttgaaggaattcacatggaggcaattctgctcagttccagagagagattcttatcatcaaaagcacacacaataaccttgcttcaccacctgccactttctccagtggcctcttgttgtgaccagtaattgagaaatgacaaatgggtatagagccaaatctctaaaacagggacaccagtgtctcctagtatctgggtaataacctcctttcagtcttagtccacaccacacactaccctccagtctctcctactctttactgtcacagaaaagactctcagcttttattcacacctgccttcagaaggccaaaccattttgtgcctgaaaactgttacccactcgccccacactttacataagtatcacatatgttctttctacaaattggtatacaggtgccatttaatccattcaaatttggaagctacatcttcaagggtctgagagagctcactccccccatatattccccctttacatgttttcttataagacatacagtttaatcaattaacaaactaaacagcttatatactggcaatatattacagatgggtttatgtcagagtaatagatcacatgaaatggaccatgtggtaccccagtgcattatgtcttggtagagccctgaggacactgacagtagcatctctaagtaagtagtgctgtatgaatacagacacatgcggatctgtatctacatccatctgactaggccaaggagcaggtagatgcaagatagagacacacacatgctggatggggccactgcacaccttgtcatgccatttaaaagggcagttacaggttgccggttttgcagccattaaaattacactttatggaaaaggcttctctaattgtgtctgatttgctttctgtagtaagcatcattggaagaagaccaaagcaagagcaactagaagttaaatatacatttgagcttagctgcaatacagaaccctggggaagaagcaggctgaaagatttatttaattttaggcttggattctctcccttgctgttttcttgatgttgtgtgtctgcatttgtgtgtgtgtgtgtgtctgcgtgtgtgtgtgttccatcacatcatctcctgaagaacgctgggtttcgcaggcaggcggctagtcacctgcaacaacccaggggtcctgccgaggcttccaggctgctgtcagtgtcagatgccagggtctggtcggtggacatggaggagatgtcattgacagacgaggatggagggagactctcactgctgttcactgctgcacctgtgctgaaggagaaggctgtccttttactacaccatttttagtcttttcttctgaattcattacttccttgtagataagttctttccattcttcaattgtgtgttctctttcatccaactgcttgtcatatatctgaggtggaggcgcctccacttcggctgggtcataccagacgttgatgtagggatgctgtaaggcgtcgtccactgatattctttttgctgggtcaatcactagcatctttgacaacaagtccctggcttggctggctttgagtttattgtgctcggagtccgctgggaagagggaatctgggaagagtttggggaaggtgagtcccgcatacttgggccgattctccacatagtttcttactgtgggttgcaatttcttcatgaattctggacatggtgttcctagttgttcaattaccttattccactggtcaatatagtcccttcctggaaagaggattttgtggcgaaccatttctcccataatgcatcccacagaccatatatccacgttctccttgtagcccatccccaggatgacctcaggggctctgtaataacgtgtcaccacatatggagtcatcatgaagcttgtgcctgctgtcctggccagtccaaagtccaggattttcaatgtgcaatcagacttgactacaatgttacttggttttaaatccctgtgaataattccagcagaatggaggtgcttaatgccacacaacatttggtacagcaggtaagacattcgctcatggtctaattccatctgaatcacttgacataagttggcatccatcagttccattactaagtaaacatcttggaactcctccagcgttttctggggtgtgaagacatttaataaactaataatgtttttatggttcacacacttcatgaggaccagctcccggtacgctctcttggcatgtgtttggttctgaaagggtctgctgagcttcttaatggccacatttctgtcaaggacagcatcatacgcggcacaaactatgccctgagccccagagccaataggctttagattctggtagcgcttgagaactgtgaaggttgagtctcccacttccacactgtagaactggttgtcaactttgcttttgctcatgttgtaatgtttggcaatatatgacacatccacttgtttatcgaatccctgtaaggaacacacacctgacaaaaggcaattttcacatccaatgttggttcactgcagtagtataagaaatggaggctcataaataccacagcttgtatggtttctcatctataggaaacgggtctaattcaacagtttcttgcataagttgccatagtgaagatctgagatgggcctgctgttggtgtttctcacactagccattccgtgcctgagaactacgatcctgatccggcagtgtttgccccagaaatcctccctacttgtttttcattaaccacattccagactaacatggaagagattctttggagatatggagattgtttaaaattaacgatggacaggtgatttccaagaaaacccaatcttaaactcactcaagcccctaggaattgaggggtgaggacaaaaaaggaaatttgtaaaaatgaaaaaagaaaagaaaaaggtaagcatatagcaagcaccacccacccccataaaaataaaaagtgaaggggaggttaaagaaaatagaagaagagtggcttgctgaatcaccctctttcactgcctggaaaccattgtgcagcgtgatgctgcctgtaccattgt

SEQ ID NO: 9217 - RNA, 4131 nt, Homo sapiens
  source 1..4131: mol_type = other RNA
agacagtagttcttgcctggtttactctgagggggaaattcaccacttatgcaggtacgagagatagcctgtcaagcactttgaagatgctggctggagacttccttctgtcttgtgatgtcatcttgcggctgatgaaattccccttgagactctctttaaagcagcttcctgctctccgcacttaatcccatgtggtataaagtaagggaggggagaagccacagatatatcaagagaaaagtaccgagaaagaaaatcagtaaagaattagagatacagagaggagaagtttttaaaaaaaaaaaaaaaaaacaggaatatgaaagagagggagctcaagtgactgaggaggcatttttaacaatcaggttatctgcaatattaaccagaaaaaaaatggtagcaaaatagagaaaatgggccatttttattccaggggacaagctgcacaaaggaatgttcttctatttattttaaacaaatgactgcgtgtactgaatctgactgtgtgaaataatctcagaatggcagcaccactggcatggcgatggtgcaggtgggtgcagttccctgtggtctctattgcttgaagagagaaagaaagttccctattattatatttaaggcagttttcagagcactggcattcttgtttgctctgttttggggatattctatttgccaatcagttcacactcatcaaccatccacttcctgtctttcacttcttcaggtgaaatatcaccactctagtgagcaccaacatggtcagagtgcaaataactgtgatggatacttcgaagtgaataagaagggaagcctgattattgctgagatcaccttggtattgccttgtacataaccaagatgtttcacagtgcctccttaagtgctcaggaaagcactttcatttaatttaatttaagctaaattctggagattttgctaaacattgacattaatgcttcatggcttttaagacaaactcatattgctaaaactatttggcagcagtaaatttatgggcagagttattgctcttacatctactgcagtacaaaactcagatgatcagcccttcgattgctcatacttattaaaataaataaataaacatgaaacatcagccacattaaggagtcagggaaactcctgaggaataacaatgtctctggagatgttttcaaatgctaacctgagactcacactgtggtttgggggtttcattattattattattattttatttcagaagaggaaagtaatattatttctcaaaataaaactttggcagagtatgaatcagggaagcagcccacacatggaaaacacaatccacaatctgaaagtagtctaggcaggctcatttttttgttgaaggaattcacatggaggcaattctgctcagttccagagagagattcttatcatcaaaagcacacacaataaccttgcttcaccacctgccactttctccagtggcctcttgttgtgaccagtaattgagaaatgacaaatgggtatagagccaaatctctaaaacagggacaccagtgtctcctagtatctgggtaataacctcctttcagtcttagtccacaccacacactaccctccagtctctcctactctttactgtcacagaaaagactctcagcttttattcacacctgccttcagaaggccaaaccattttgtgcctgaaaactgttacccactcgccccacactttacataagtatcacatatgttctttctacaaattggtatacaggtgccatttaatccattcaaatttggaagctacatcttcaagggtctgagagagctcactccccccatatattccccctttacatgttttcttataagacatacagtttaatcaattaacaaactaaacagcttatatactggcaatatattacagatgggtttatgtcagagtaatagatcacatgaaatggaccatgtggtaccccagtgcattatgtcttggtagagccctgaggacactgacagtagcatctctaagtaagtagtgctgtatgaatacagacacatgcggatctgtatctacatccatctgactaggccaaggagcaggtagatgcaagatagagacacacacatgctggatggggccactgcacaccttgtcatgccatttaaaagggcagttacaggttgccggttttgcagccattaaaattacactttatggaaaaggcttctctaattgtgtctgatttgctttctgtagtaagcatcattggaagaagaccaaagcaagagcaactagaagttaaatatacatttgagcttagctgcaatacagaaccctggggaagaagcaggctgaaagatttatttaattttaggcttggattctctcccttgctgttttcttgatgttgtgtgtctgcatttgtgtgtgtgtgtgtgtctgcgtgtgtgtgtgttccatcacatcatctcctgaagaacgctgggtttcgcaggcaggcggctagtcacctgcaacaacccaggggtcctgccgaggcttccaggctgctgtcagtgtcagatgccagggtctggtcggtggacatggaggagatgtcattgacagacgaggatggagggagactctcactgctgttcactgctgcacctgtgctgaaggagaaggctgtccttttactacaccatttttagtcttttcttctgaattcattacttccttgtagataagttctttccattcttcaattgtgtgttctctttcatccaactgcttgtcatatatctgaggtggaggcgcctccacttcggctgggtcataccagacgttgatgtagggatgctgtaaggcgtcgtccactgatattctttttgctgggtcaatcactagcatctttgacaacaagtccctggcttggctggctttgagtttattgtgctcggagtccgctgggaagagggaatctgggaagagtttggggaaggtgagtcccgcatacttgggccgattctccacatagtttcttactgtgggttgcaatttcttcatgaattctggacatggtgttcctagttgttcaattaccttattccactggtcaatatagtcccttcctggaaagaggattttgtggcgaaccatttctcccataatgcatcccacagaccatatatccacgttctccttgtagcccatccccaggatgacctcaggggctctgtaataacgtgtcaccacatatggagtcatcatgaagcttgtgcctgctgtcctggccagtccaaagtccaggattttcaatgtgcaatcagacttgactacaatgttacttggttttaaatccctgtgaataattccagcagaatggaggtgcttaatgccacacaacatttggtacagcaggtaagacattcgctcatggtctaattccatctgaatcacttgacataagttggcatccatcagttccattactaagtaaacatcttggaactcctccagcgttttctggggtgtgaagacatttaataaactaataatgtttttatggttcacacacttcatgaggaccagctcccggtacgctctcttggcatgtgtttggttctgaaagggtctgctgagcttcttaatggccacatttctgtcaaggacagcatcatacgcggcacaaactatgccctgagccccagagccaataggctttagattctggtagcgcttgagaactgtgaaggttgagtctcccacttccacactgtagaactggttgtcaactttgcttttgctcatgttgtaatgtttggcaatatatgacacatccacttgtttatcgaatcccttgttttacctgtaaggaacacacacctgacaaaaggcaattttcacatccaatgttggttcactgcagtagtataagaaatggaggctcataaataccacagcttgtatggtttctcatctataggaaacgggtctaattcaacagtttcttgcataagttgccatagtgaagatctgagatgggcctgctgttggtgtttctcacactagccagacaatgacagcaaaaacacactcagcccctctgggatctgttcataaacatccccttccagcat

SEQ ID NO: 9218 - RNA, 4114 nt, Homo sapiens
  source 1..4114: mol_type = other RNA
agacagtagttcttgcctggtttactctgagggggaaattcaccacttatgcaggtacgagagatagcctgtcaagcactttgaagatgctggctggagacttccttctgtcttgtgatgtcatcttgcggctgatgaaattccccttgagactctctttaaagcagcttcctgctctccgcacttaatcccatgtggtataaagtaagggaggggagaagccacagatatatcaagagaaaagtaccgagaaagaaaatcagtaaagaattagagatacagagaggagaagtttttaaaaaaaaaaaaaaaaaacaggaatatgaaagagagggagctcaagtgactgaggaggcatttttaacaatcaggttatctgcaatattaaccagaaaaaaaatggtagcaaaatagagaaaatgggccatttttattccaggggacaagctgcacaaaggaatgttcttctatttattttaaacaaatgactgcgtgtactgaatctgactgtgtgaaataatctcagaatggcagcaccactggcatggcgatggtgcaggtgggtgcagttccctgtggtctctattgcttgaagagagaaagaaagttccctattattatatttaaggcagttttcagagcactggcattcttgtttgctctgttttggggatattctatttgccaatcagttcacactcatcaaccatccacttcctgtctttcacttcttcaggtgaaatatcaccactctagtgagcaccaacatggtcagagtgcaaataactgtgatggatacttcgaagtgaataagaagggaagcctgattattgctgagatcaccttggtattgccttgtacataaccaagatgtttcacagtgcctccttaagtgctcaggaaagcactttcatttaatttaatttaagctaaattctggagattttgctaaacattgacattaatgcttcatggcttttaagacaaactcatattgctaaaactatttggcagcagtaaatttatgggcagagttattgctcttacatctactgcagtacaaaactcagatgatcagcccttcgattgctcatacttattaaaataaataaataaacatgaaacatcagccacattaaggagtcagggaaactcctgaggaataacaatgtctctggagatgttttcaaatgctaacctgagactcacactgtggtttgggggtttcattattattattattattttatttcagaagaggaaagtaatattatttctcaaaataaaactttggcagagtatgaatcagggaagcagcccacacatggaaaacacaatccacaatctgaaagtagtctaggcaggctcatttttttgttgaaggaattcacatggaggcaattctgctcagttccagagagagattcttatcatcaaaagcacacacaataaccttgcttcaccacctgccactttctccagtggcctcttgttgtgaccagtaattgagaaatgacaaatgggtatagagccaaatctctaaaacagggacaccagtgtctcctagtatctgggtaataacctcctttcagtcttagtccacaccacacactaccctccagtctctcctactctttactgtcacagaaaagactctcagcttttattcacacctgccttcagaaggccaaaccattttgtgcctgaaaactgttacccactcgccccacactttacataagtatcacatatgttctttctacaaattggtatacaggtgccatttaatccattcaaatttggaagctacatcttcaagggtctgagagagctcactccccccatatattccccctttacatgttttcttataagacatacagtttaatcaattaacaaactaaacagcttatatactggcaatatattacagatgggtttatgtcagagtaatagatcacatgaaatggaccatgtggtaccccagtgcattatgtcttggtagagccctgaggacactgacagtagcatctctaagtaagtagtgctgtatgaatacagacacatgcggatctgtatctacatccatctgactaggccaaggagcaggtagatgcaagatagagacacacacatgctggatggggccactgcacaccttgtcatgccatttaaaagggcagttacaggttgccggttttgcagccattaaaattacactttatggaaaaggcttctctaattgtgtctgatttgctttctgtagtaagcatcattggaagaagaccaaagcaagagcaactagaagttaaatatacatttgagcttagctgcaatacagaaccctggggaagaagcaggctgaaagatttatttaattttaggcttggattctctcccttgctgttttcttgatgttgtgtgtctgcatttgtgtgtgtgtgtgtgtctgcgtgtgtgtgtgttccatcacatcatctcctgaagaacgctgggtttcgcaggcaggcggctagtcacctgcaacaacccaggggtcctgccgaggcttccaggctgctgtcagtgtcagatgccagggtctggtcggtggacatggaggagatgtcattgacagacgaggatggagggagactctcactgctgttcactgctgcacctgtgctgaaggagaaggctgtccttttactacaccatttttagtcttttcttctgaattcattacttccttgtagataagttctttccattcttcaattgtgtgttctctttcatccaactgcttgtcatatatctgaggtggaggcgcctccacttcggctgggtcataccagacgttgatgtagggatgctgtaaggcgtcgtccactgatattctttttgctgggtcaatcactagcatctttgacaacaagtccctggcttggctggctttgagtttattgtgctcggagtccgctgggaagagggaatctgggaagagtttggggaaggtgagtcccgcatacttgggccgattctccacatagtttcttactgtgggttgcaatttcttcatgaattctggacatggtgttcctagttgttcaattaccttattccactggtcaatatagtcccttcctggaaagaggattttgtggcgaaccatttctcccataatgcatcccacagaccatatatccacgttctccttgtagcccatccccaggatgacctcaggggctctgtaataacgtgtcaccacatatggagtcatcatgaagcttgtgcctgctgtcctggccagtccaaagtccaggattttcaatgtgcaatcagacttgactacaatgttacttggttttaaatccctgtgaataattccagcagaatggaggtgcttaatgccacacaacatttggtacagcaggtaagacattcgctcatggtctaattccatctgaatcacttgacataagttggcatccatcagttccattactaagtaaacatcttggaactcctccagcgttttctggggtgtgaagacatttaataaactaataatgtttttatggttcacacacttcatgaggaccagctcccggtacgctctcttggcatgtgtttggttctgaaagggtctgctgagcttcttaatggccacatttctgtcaaggacagcatcatacgcggcacaaactatgccctgagccccagagccaataggctttagattctggtagcgcttgagaactgtgaaggttgagtctcccacttccacactgtagaactggttgtcaactttgcttttgctcatgttgtaatgtttggcaatatatgacacatccacttgtttatcgaatcccttgttttacctgtaaggaacacacacctgacaaaaggcaattttcacatccaatgttggttcactgcagtagtataagaaatggaggctcataaataccacagcttgtatggtttctcatctataggaaacgggtctaattcaacagtttcttgcataagttgccatagtgaagatctgagatgggcctgctgttggtgtttctcacactagccagaggcagccaaaccgctacatccaaagcatccagcccctaaaatctaa

SEQ ID NO: 9219 - RNA, 4467 nt, Homo sapiens
  source 1..4467: mol_type = other RNA
agacagtagttcttgcctggtttactctgagggggaaattcaccacttatgcaggtacgagagatagcctgtcaagcactttgaagatgctggctggagacttccttctgtcttgtgatgtcatcttgcggctgatgaaattccccttgagactctctttaaagcagcttcctgctctccgcacttaatcccatgtggtataaagtaagggaggggagaagccacagatatatcaagagaaaagtaccgagaaagaaaatcagtaaagaattagagatacagagaggagaagtttttaaaaaaaaaaaaaaaaaacaggaatatgaaagagagggagctcaagtgactgaggaggcatttttaacaatcaggttatctgcaatattaaccagaaaaaaaatggtagcaaaatagagaaaatgggccatttttattccaggggacaagctgcacaaaggaatgttcttctatttattttaaacaaatgactgcgtgtactgaatctgactgtgtgaaataatctcagaatggcagcaccactggcatggcgatggtgcaggtgggtgcagttccctgtggtctctattgcttgaagagagaaagaaagttccctattattatatttaaggcagttttcagagcactggcattcttgtttgctctgttttggggatattctatttgccaatcagttcacactcatcaaccatccacttcctgtctttcacttcttcaggtgaaatatcaccactctagtgagcaccaacatggtcagagtgcaaataactgtgatggatacttcgaagtgaataagaagggaagcctgattattgctgagatcaccttggtattgccttgtacataaccaagatgtttcacagtgcctccttaagtgctcaggaaagcactttcatttaatttaatttaagctaaattctggagattttgctaaacattgacattaatgcttcatggcttttaagacaaactcatattgctaaaactatttggcagcagtaaatttatgggcagagttattgctcttacatctactgcagtacaaaactcagatgatcagcccttcgattgctcatacttattaaaataaataaataaacatgaaacatcagccacattaaggagtcagggaaactcctgaggaataacaatgtctctggagatgttttcaaatgctaacctgagactcacactgtggtttgggggtttcattattattattattattttatttcagaagaggaaagtaatattatttctcaaaataaaactttggcagagtatgaatcagggaagcagcccacacatggaaaacacaatccacaatctgaaagtagtctaggcaggctcatttttttgttgaaggaattcacatggaggcaattctgctcagttccagagagagattcttatcatcaaaagcacacacaataaccttgcttcaccacctgccactttctccagtggcctcttgttgtgaccagtaattgagaaatgacaaatgggtatagagccaaatctctaaaacagggacaccagtgtctcctagtatctgggtaataacctcctttcagtcttagtccacaccacacactaccctccagtctctcctactctttactgtcacagaaaagactctcagcttttattcacacctgccttcagaaggccaaaccattttgtgcctgaaaactgttacccactcgccccacactttacataagtatcacatatgttctttctacaaattggtatacaggtgccatttaatccattcaaatttggaagctacatcttcaagggtctgagagagctcactccccccatatattccccctttacatgttttcttataagacatacagtttaatcaattaacaaactaaacagcttatatactggcaatatattacagatgggtttatgtcagagtaatagatcacatgaaatggaccatgtggtaccccagtgcattatgtcttggtagagccctgaggacactgacagtagcatctctaagtaagtagtgctgtatgaatacagacacatgcggatctgtatctacatccatctgactaggccaaggagcaggtagatgcaagatagagacacacacatgctggatggggccactgcacaccttgtcatgccatttaaaagggcagttacaggttgccggttttgcagccattaaaattacactttatggaaaaggcttctctaattgtgtctgatttgctttctgtagtaagcatcattggaagaagaccaaagcaagagcaactagaagttaaatatacatttgagcttagctgcaatacagaaccctggggaagaagcaggctgaaagatttatttaattttaggcttggattctctcccttgctgttttcttgatgttgtgtgtctgcatttgtgtgtgtgtgtgtgtctgcgtgtgtgtgtgttccatcacatcatctcctgaagaacgctgggtttcgcaggcaggcggctagtcacctgcaacaacccaggggtcctgccgaggcttccaggctgctgtcagtgtcagatgccagggtctggtcggtggacatggaggagatgtcattgacagacgaggatggagggagactctcactgctgttcactgctgcacctgtgctgaaggagaaggctgtccttttactacaccatttttagtcttttcttctgaattcattacttccttgtagataagttctttccattcttcaattgtgtgttctctttcatccaactgcttgtcatatatctgaggtggaggcgcctccacttcggctgggtcataccagacgttgatgtagggatgctgtaaggcgtcgtccactgatattctttttgctgggtcaatcactagcatctttgacaacaagtccctggcttggctggctttgagtttattgtgctcggagtccgctgggaagagggaatctgggaagagtttggggaaggtgagtcccgcatacttgggccgattctccacatagtttcttactgtgggttgcaatttcttcatgaattctggacatggtgttcctagttgttcaattaccttattccactggtcaatatagtcccttcctggaaagaggattttgtggcgaaccatttctcccataatgcatcccacagaccatatatccacgttctccttgtagcccatccccaggatgacctcaggggctctgtaataacgtgtcaccacatatggagtcatcatgaagcttgtgcctgctgtcctggccagtccaaagtccaggattttcaatgtgcaatcagacttgactacaatgttacttggttttaaatccctgtgaataattccagcagaatggaggtgcttaatgccacacaacatttggtacagcaggtaagacattcgctcatggtctaattccatctgaatcacttgacataagttggcatccatcagttccattactaagtaaacatcttggaactcctccagcgttttctggggtgtgaagacatttaataaactaataatgtttttatggttcacacacttcatgaggaccagctcccggtacgctctcttggcatgtgtttggttctgaaagggtctgctgagcttcttaatggccacatttctgtcaaggacagcatcatacgcggcacaaactatgccctgagccccagagccaataggctttagattctggtagcgcttgagaactgtgaaggttgagtctcccacttccacactgtagaactggttgtcaactttgcttttgctcatgttgtaatgtttggcaatatatgacacatccacttgtttatcgaatcccttgttttacctgtaaggaacacacacctgacaaaaggcaattttcacatccaatgttggttcactgcagtagtataagaaatggaggctcataaataccacagcttgtatggtttctcatctataggaaacgggtctaattcaacagtttcttgcataagttgccatagtgaagatctgagatgggcctgctgttggtgtttctcacactagccattccgtgcctgagaactacgatcctgatccggcagtgtttgccccagaaatcctccctacttgtttttcattaaccacattccagactaacatggaagagattctttggagatatggagattgtttaaaattaacgatggacaggtgatttccaagaaaacccaatcttaaactcactcaagcccctaggaattgaggggtgaggacaaaaaaggaaatttgtaaaaatgaaaaaagaaaagaaaaaggtaagcatatagcaagcaccacccacccccataaaaataaaaagtgaaggggaggttaaagaaaatagaagaagagtggcttgctgaatcaccctctttcactgcctggaaaccattgtgcagcgtgatgctgcctgtaccattgtggaacct

SEQ ID NO: 9220 - RNA, 4369 nt, Homo sapiens
  source 1..4369: mol_type = other RNA
agacagtagttcttgcctggtttactctgagggggaaattcaccacttatgcaggtacgagagatagcctgtcaagcactttgaagatgctggctggagacttccttctgtcttgtgatgtcatcttgcggctgatgaaattccccttgagactctctttaaagcagcttcctgctctccgcacttaatcccatgtggtataaagtaagggaggggagaagccacagatatatcaagagaaaagtaccgagaaagaaaatcagtaaagaattagagatacagagaggagaagtttttaaaaaaaaaaaaaaaaaacaggaatatgaaagagagggagctcaagtgactgaggaggcatttttaacaatcaggttatctgcaatattaaccagaaaaaaaatggtagcaaaatagagaaaatgggccatttttattccaggggacaagctgcacaaaggaatgttcttctatttattttaaacaaatgactgcgtgtactgaatctgactgtgtgaaataatctcagaatggcagcaccactggcatggcgatggtgcaggtgggtgcagttccctgtggtctctattgcttgaagagagaaagaaagttccctattattatatttaaggcagttttcagagcactggcattcttgtttgctctgttttggggatattctatttgccaatcagttcacactcatcaaccatccacttcctgtctttcacttcttcaggtgaaatatcaccactctagtgagcaccaacatggtcagagtgcaaataactgtgatggatacttcgaagtgaataagaagggaagcctgattattgctgagatcaccttggtattgccttgtacataaccaagatgtttcacagtgcctccttaagtgctcaggaaagcactttcatttaatttaatttaagctaaattctggagattttgctaaacattgacattaatgcttcatggcttttaagacaaactcatattgctaaaactatttggcagcagtaaatttatgggcagagttattgctcttacatctactgcagtacaaaactcagatgatcagcccttcgattgctcatacttattaaaataaataaataaacatgaaacatcagccacattaaggagtcagggaaactcctgaggaataacaatgtctctggagatgttttcaaatgctaacctgagactcacactgtggtttgggggtttcattattattattattattttatttcagaagaggaaagtaatattatttctcaaaataaaactttggcagagtatgaatcagggaagcagcccacacatggaaaacacaatccacaatctgaaagtagtctaggcaggctcatttttttgttgaaggaattcacatggaggcaattctgctcagttccagagagagattcttatcatcaaaagcacacacaataaccttgcttcaccacctgccactttctccagtggcctcttgttgtgaccagtaattgagaaatgacaaatgggtatagagccaaatctctaaaacagggacaccagtgtctcctagtatctgggtaataacctcctttcagtcttagtccacaccacacactaccctccagtctctcctactctttactgtcacagaaaagactctcagcttttattcacacctgccttcagaaggccaaaccattttgtgcctgaaaactgttacccactcgccccacactttacataagtatcacatatgttctttctacaaattggtatacaggtgccatttaatccattcaaatttggaagctacatcttcaagggtctgagagagctcactccccccatatattccccctttacatgttttcttataagacatacagtttaatcaattaacaaactaaacagcttatatactggcaatatattacagatgggtttatgtcagagtaatagatcacatgaaatggaccatgtggtaccccagtgcattatgtcttggtagagccctgaggacactgacagtagcatctctaagtaagtagtgctgtatgaatacagacacatgcggatctgtatctacatccatctgactaggccaaggagcaggtagatgcaagatagagacacacacatgctggatggggccactgcacaccttgtcatgccatttaaaagggcagttacaggttgccggttttgcagccattaaaattacactttatggaaaaggcttctctaattgtgtctgatttgctttctgtagtaagcatcattggaagaagaccaaagcaagagcaactagaagttaaatatacatttgagcttagctgcaatacagaaccctggggaagaagcaggctgaaagatttatttaattttaggcttggattctctcccttgctgttttcttgatgttgtgtgtctgcatttgtgtgtgtgtgtgtgtctgcgtgtgtgtgtgttccatcacatcatctcctgaagaacgctgggtttcgcaggcaggcggctagtcacctgcaacaacccaggggtcctgccgaggcttccaggctgctgtcagtgtcagatgccagggtctggtcggtggacatggaggagatgtcattgacagacgaggatggagggagactctcactgctgttcactgctgcacctgtgctgaaggagaaggctgtccttttactacaccatttttagtcttttcttctgaattcattacttccttgtagataagttctttccattcttcaattgtgtgttctctttcatccaactgcttgtcatatatctgaggtggaggcgcctccacttcggctgggtcataccagacgttgatgtagggatgctgtaaggcgtcgtccactgatattctttttgctgggtcaatcactagcatctttgacaacaagtccctggcttggctggctttgagtttattgtgctcggagtccgctgggaagagggaatctgggaagagtttggggaaggtgagtcccgcatacttgggccgattctccacatagtttcttactgtgggttgcaatttcttcatgaattctggacatggtgttcctagttgttcaattaccttattccactggtcaatatagtcccttcctggaaagaggattttgtggcgaaccatttctcccataatgcatcccacagaccatatatccacgttctccttgtagcccatccccaggatgacctcaggggctctgtaataacgtgtcaccacatatggagtcatcatgaagcttgtgcctgctgtcctggccagtccaaagtccaggattttcaatgtgcaatcagacttgactacaatgttacttggttttaaatccctgtgaataattccagcagaatggaggtgcttaatgccacacaacatttggtacagcaggtaagacattcgctcatggtctaattccatctgaatcacttgacataagttggcatccatcagttccattactaagtaaacatcttggaactcctccagcgttttctggggtgtgaagacatttaataaactaataatgtttttatggttcacacacttcatgaggaccagctcccggtacgctctcttggcatgtgtttggttctgaaagggtctgctgagcttcttaatggccacatttctgtcaaggacagcatcatacgcggcacaaactatgccctgagccccagagccaataggctttagattctggtagcgcttgagaactgtgaaggttgagtctcccacttccacactgtagaactggttgtcaactttgcttttgctcatgttgtaatgtttggcaatatatgacacatccacttgtttatcgaatcccttgttttacctgtaaggaacacacacctgacaaaaggcaattttcacatccaatgttggttcactgcagtagtataagaaatggaggctcataaataccacagcttgtatggtttctcatctataggaaacgggtctaattcaacagtttcttgcataagttgccatagtgaagatctgagatgggcctgctgttggtgtttctcacactagcctaaagtagaaaattcacagaagcttctctgagagaaatggtccttactgcaactattttaaatatgttgataagcattctgtgttatcttccagggtccgacaactagccgatgagggatagaaggagatattggatgttgtgctggcaatgcctggtgcacttacactcgttttccttccacctgaactgtagtctatcccatatgacttagcctgcttccttgcagtttgttcataaaagttatcatcaacatggccagaagcaggcagggctgctgtacagacactgtcaggctctgcacc

SEQ ID NO: 9221 - RNA, 4263 nt, Homo sapiens
  source 1..4263: mol_type = other RNA
agacagtagttcttgcctggtttactctgagggggaaattcaccacttatgcaggtacgagagatagcctgtcaagcactttgaagatgctggctggagacttccttctgtcttgtgatgtcatcttgcggctgatgaaattccccttgagactctctttaaagcagcttcctgctctccgcacttaatcccatgtggtataaagtaagggaggggagaagccacagatatatcaagagaaaagtaccgagaaagaaaatcagtaaagaattagagatacagagaggagaagtttttaaaaaaaaaaaaaaaaaacaggaatatgaaagagagggagctcaagtgactgaggaggcatttttaacaatcaggttatctgcaatattaaccagaaaaaaaatggtagcaaaatagagaaaatgggccatttttattccaggggacaagctgcacaaaggaatgttcttctatttattttaaacaaatgactgcgtgtactgaatctgactgtgtgaaataatctcagaatggcagcaccactggcatggcgatggtgcaggtgggtgcagttccctgtggtctctattgcttgaagagagaaagaaagttccctattattatatttaaggcagttttcagagcactggcattcttgtttgctctgttttggggatattctatttgccaatcagttcacactcatcaaccatccacttcctgtctttcacttcttcaggtgaaatatcaccactctagtgagcaccaacatggtcagagtgcaaataactgtgatggatacttcgaagtgaataagaagggaagcctgattattgctgagatcaccttggtattgccttgtacataaccaagatgtttcacagtgcctccttaagtgctcaggaaagcactttcatttaatttaatttaagctaaattctggagattttgctaaacattgacattaatgcttcatggcttttaagacaaactcatattgctaaaactatttggcagcagtaaatttatgggcagagttattgctcttacatctactgcagtacaaaactcagatgatcagcccttcgattgctcatacttattaaaataaataaataaacatgaaacatcagccacattaaggagtcagggaaactcctgaggaataacaatgtctctggagatgttttcaaatgctaacctgagactcacactgtggtttgggggtttcattattattattattattttatttcagaagaggaaagtaatattatttctcaaaataaaactttggcagagtatgaatcagggaagcagcccacacatggaaaacacaatccacaatctgaaagtagtctaggcaggctcatttttttgttgaaggaattcacatggaggcaattctgctcagttccagagagagattcttatcatcaaaagcacacacaataaccttgcttcaccacctgccactttctccagtggcctcttgttgtgaccagtaattgagaaatgacaaatgggtatagagccaaatctctaaaacagggacaccagtgtctcctagtatctgggtaataacctcctttcagtcttagtccacaccacacactaccctccagtctctcctactctttactgtcacagaaaagactctcagcttttattcacacctgccttcagaaggccaaaccattttgtgcctgaaaactgttacccactcgccccacactttacataagtatcacatatgttctttctacaaattggtatacaggtgccatttaatccattcaaatttggaagctacatcttcaagggtctgagagagctcactccccccatatattccccctttacatgttttcttataagacatacagtttaatcaattaacaaactaaacagcttatatactggcaatatattacagatgggtttatgtcagagtaatagatcacatgaaatggaccatgtggtaccccagtgcattatgtcttggtagagccctgaggacactgacagtagcatctctaagtaagtagtgctgtatgaatacagacacatgcggatctgtatctacatccatctgactaggccaaggagcaggtagatgcaagatagagacacacacatgctggatggggccactgcacaccttgtcatgccatttaaaagggcagttacaggttgccggttttgcagccattaaaattacactttatggaaaaggcttctctaattgtgtctgatttgctttctgtagtaagcatcattggaagaagaccaaagcaagagcaactagaagttaaatatacatttgagcttagctgcaatacagaaccctggggaagaagcaggctgaaagatttatttaattttaggcttggattctctcccttgctgttttcttgatgttgtgtgtctgcatttgtgtgtgtgtgtgtgtctgcgtgtgtgtgtgttccatcacatcatctcctgaagaacgctgggtttcgcaggcaggcggctagtcacctgcaacaacccaggggtcctgccgaggcttccaggctgctgtcagtgtcagatgccagggtctggtcggtggacatggaggagatgtcattgacagacgaggatggagggagactctcactgctgttcactgctgcacctgtgctgaaggagaaggctgtccttttactacaccatttttagtcttttcttctgaattcattacttccttgtagataagttctttccattcttcaattgtgtgttctctttcatccaactgcttgtcatatatctgaggtggaggcgcctccacttcggctgggtcataccagacgttgatgtagggatgctgtaaggcgtcgtccactgatattctttttgctgggtcaatcactagcatctttgacaacaagtccctggcttggctggctttgagtttattgtgctcggagtccgctgggaagagggaatctgggaagagtttggggaaggtgagtcccgcatacttgggccgattctccacatagtttcttactgtgggttgcaatttcttcatgaattctggacatggtgttcctagttgttcaattaccttattccactggtcaatatagtcccttcctggaaagaggattttgtggcgaaccatttctcccataatgcatcccacagaccatatatccacgttctccttgtagcccatccccaggatgacctcaggggctctgtaataacgtgtcaccacatatggagtcatcatgaagcttgtgcctgctgtcctggccagtccaaagtccaggattttcaatgtgcaatcagacttgactacaatgttacttggttttaaatccctgtgaataattccagcagaatggaggtgcttaatgccacacaacatttggtacagcaggtaagacattcgctcatggtctaattccatctgaatcacttgacataagttggcatccatcagttccattactaagtaaacatcttggaactcctccagcgttttctggggtgtgaagacatttaataaactaataatgtttttatggttcacacacttcatgaggaccagctcccggtacgctctcttggcatgtgtttggttctgaaagggtctgctgagcttcttaatggccacatttctgtcaaggacagcatcatacgcggcactgacaaaaggcaattttcacatccaatgttggttcactgcagtagtataagaaatggaggctcataaataccacagcttgtatggtttctcatctataggaaacgggtctaattcaacagtttcttgcataagttgccatagtgaagatctgagatgggcctgctgttggtgtttctcacactagccattccgtgcctgagaactacgatcctgatccggcagtgtttgccccagaaatcctccctacttgtttttcattaaccacattccagactaacatggaagagattctttggagatatggagattgtttaaaattaacgatggacaggtgatttccaagaaaacccaatcttaaactcactcaagcccctaggaattgaggggtgaggacaaaaaaggaaatttgtaaaaatgaaaaaagaaaagaaaaaggtaagcatatagcaagcaccacccacccccataaaaataaaaagtgaaggggaggttaaagaaaatagaagaagagtggcttgctgaatcaccctctttcactgcctggaaaccattgtgcagcgtgatgctgcctgtaccattgt

SEQ ID NO: 9222 - RNA, 4401 nt, Homo sapiens
  source 1..4401: mol_type = other RNA
agacagtagttcttgcctggtttactctgagggggaaattcaccacttatgcaggtacgagagatagcctgtcaagcactttgaagatgctggctggagacttccttctgtcttgtgatgtcatcttgcggctgatgaaattccccttgagactctctttaaagcagcttcctgctctccgcacttaatcccatgtggtataaagtaagggaggggagaagccacagatatatcaagagaaaagtaccgagaaagaaaatcagtaaagaattagagatacagagaggagaagtttttaaaaaaaaaaaaaaaaaacaggaatatgaaagagagggagctcaagtgactgaggaggcatttttaacaatcaggttatctgcaatattaaccagaaaaaaaatggtagcaaaatagagaaaatgggccatttttattccaggggacaagctgcacaaaggaatgttcttctatttattttaaacaaatgactgcgtgtactgaatctgactgtgtgaaataatctcagaatggcagcaccactggcatggcgatggtgcaggtgggtgcagttccctgtggtctctattgcttgaagagagaaagaaagttccctattattatatttaaggcagttttcagagcactggcattcttgtttgctctgttttggggatattctatttgccaatcagttcacactcatcaaccatccacttcctgtctttcacttcttcaggtgaaatatcaccactctagtgagcaccaacatggtcagagtgcaaataactgtgatggatacttcgaagtgaataagaagggaagcctgattattgctgagatcaccttggtattgccttgtacataaccaagatgtttcacagtgcctccttaagtgctcaggaaagcactttcatttaatttaatttaagctaaattctggagattttgctaaacattgacattaatgcttcatggcttttaagacaaactcatattgctaaaactatttggcagcagtaaatttatgggcagagttattgctcttacatctactgcagtacaaaactcagatgatcagcccttcgattgctcatacttattaaaataaataaataaacatgaaacatcagccacattaaggagtcagggaaactcctgaggaataacaatgtctctggagatgttttcaaatgctaacctgagactcacactgtggtttgggggtttcattattattattattattttatttcagaagaggaaagtaatattatttctcaaaataaaactttggcagagtatgaatcagggaagcagcccacacatggaaaacacaatccacaatctgaaagtagtctaggcaggctcatttttttgttgaaggaattcacatggaggcaattctgctcagttccagagagagattcttatcatcaaaagcacacacaataaccttgcttcaccacctgccactttctccagtggcctcttgttgtgaccagtaattgagaaatgacaaatgggtatagagccaaatctctaaaacagggacaccagtgtctcctagtatctgggtaataacctcctttcagtcttagtccacaccacacactaccctccagtctctcctactctttactgtcacagaaaagactctcagcttttattcacacctgccttcagaaggccaaaccattttgtgcctgaaaactgttacccactcgccccacactttacataagtatcacatatgttctttctacaaattggtatacaggtgccatttaatccattcaaatttggaagctacatcttcaagggtctgagagagctcactccccccatatattccccctttacatgttttcttataagacatacagtttaatcaattaacaaactaaacagcttatatactggcaatatattacagatgggtttatgtcagagtaatagatcacatgaaatggaccatgtggtaccccagtgcattatgtcttggtagagccctgaggacactgacagtagcatctctaagtaagtagtgctgtatgaatacagacacatgcggatctgtatctacatccatctgactaggccaaggagcaggtagatgcaagatagagacacacacatgctggatggggccactgcacaccttgtcatgccatttaaaagggcagttacaggttgccggttttgcagccattaaaattacactttatggaaaaggcttctctaattgtgtctgatttgctttctgtagtaagcatcattggaagaagaccaaagcaagagcaactagaagttaaatatacatttgagcttagctgcaatacagaaccctggggaagaagcaggctgaaagatttatttaattttaggcttggattctctcccttgctgttttcttgatgttgtgtgtctgcatttgtgtgtgtgtgtgtgtctgcgtgtgtgtgtgttccatcacatcatctcctgaagaacgctgggtttcgcaggcaggcggctagtcacctgcaacaacccaggggtcctgccgaggcttccaggctgctgtcagtgtcagatgccagggtctggtcggtggacatggaggagatgtcattgacagacgaggatggagggagactctcactgctgttcactgctgcacctgtgctgaaggagaaggctgtccttttactacaccatttttagtcttttcttctgaattcattacttccttgtagataagttctttccattcttcaattgtgtgttctctttcatccaactgcttgtcatatatctgaggtggaggcgcctccacttcggctgggtcataccagacgttgatgtagggatgctgtaaggcgtcgtccactgatattctttttgctgggtcaatcactagcatctttgacaacaagtccctggcttggctggctttgagtttattgtgctcggagtccgctgggaagagggaatctgggaagagtttggggaaggtgagtcccgcatacttgggccgattctccacatagtttcttactgtgggttgcaatttcttcatgaattctggacatggtgttcctagttgttcaattaccttattccactggtcaatatagtcccttcctggaaagaggattttgtggcgaaccatttctcccataatgcatcccacagaccatatatccacgttctccttgtagcccatccccaggatgacctcaggggctctgtaataacgtgtcaccacatatggagtcatcatgaagcttgtgcctgctgtcctggccagtccaaagtccaggattttcaatgtgcaatcagacttgactacaatgttacttggttttaaatccctgtgaataattccagcagaatggaggtgcttaatgccacacaacatttggtacagcaggtaagacattcgctcatggtctaattccatctgaatcacttgacataagttggcatccatcagttccattactaagtaagtttttatggttcacacacttcatgaggaccagctcccggtacgctctcttggcatgtgtttggttctgaaagggtctgctgagcttcttaatggccacatttctgtcaaggacagcatcatacgcggcacaaactatgccctgagccccagagccaataggctttagattctggtagcgcttgagaactgtgaaggttgagtctcccacttccacactgtagaactggttgtcaactttgcttttgctcatgttgtaatgtttggcaatatatgacacatccacttgtttatcgaatcccttgttttacctgtaaggaacacacacctgacaaaaggcaattttcacatccaatgttggttcactgcagtagtataagaaatggaggctcataaataccacagcttgtatggtttctcatctataggaaacgggtctaattcaacagtttcttgcataagttgccatagtgaagatctgagatgggcctgctgttggtgtttctcacactagccattccgtgcctgagaactacgatcctgatccggcagtgtttgccccagaaatcctccctacttgtttttcattaaccacattccagactaacatggaagagattctttggagatatggagattgtttaaaattaacgatggacaggtgatttccaagaaaacccaatcttaaactcactcaagcccctaggaattgaggggtgaggacaaaaaaggaaatttgtaaaaatgaaaaaagaaaagaaaaaggtaagcatatagcaagcaccacccacccccataaaaataaaaagtgaaggggaggttaaagaaaatagaagaagagtggcttgctgaatcaccctctttcactgcctggaaaccattgtgcagcgtgatgctgcctgtaccattgt

SEQ ID NO: 9223 - RNA, 4389 nt, Homo sapiens
  source 1..4389: mol_type = other RNA
agacagtagttcttgcctggtttactctgagggggaaattcaccacttatgcaggtacgagagatagcctgtcaagcactttgaagatgctggctggagacttccttctgtcttgtgatgtcatcttgcggctgatgaaattccccttgagactctctttaaagcagcttcctgctctccgcacttaatcccatgtggtataaagtaagggaggggagaagccacagatatatcaagagaaaagtaccgagaaagaaaatcagtaaagaattagagatacagagaggagaagtttttaaaaaaaaaaaaaaaaaacaggaatatgaaagagagggagctcaagtgactgaggaggcatttttaacaatcaggttatctgcaatattaaccagaaaaaaaatggtagcaaaatagagaaaatgggccatttttattccaggggacaagctgcacaaaggaatgttcttctatttattttaaacaaatgactgcgtgtactgaatctgactgtgtgaaataatctcagaatggcagcaccactggcatggcgatggtgcaggtgggtgcagttccctgtggtctctattgcttgaagagagaaagaaagttccctattattatatttaaggcagttttcagagcactggcattcttgtttgctctgttttggggatattctatttgccaatcagttcacactcatcaaccatccacttcctgtctttcacttcttcaggtgaaatatcaccactctagtgagcaccaacatggtcagagtgcaaataactgtgatggatacttcgaagtgaataagaagggaagcctgattattgctgagatcaccttggtattgccttgtacataaccaagatgtttcacagtgcctccttaagtgctcaggaaagcactttcatttaatttaatttaagctaaattctggagattttgctaaacattgacattaatgcttcatggcttttaagacaaactcatattgctaaaactatttggcagcagtaaatttatgggcagagttattgctcttacatctactgcagtacaaaactcagatgatcagcccttcgattgctcatacttattaaaataaataaataaacatgaaacatcagccacattaaggagtcagggaaactcctgaggaataacaatgtctctggagatgttttcaaatgctaacctgagactcacactgtggtttgggggtttcattattattattattattttatttcagaagaggaaagtaatattatttctcaaaataaaactttggcagagtatgaatcagggaagcagcccacacatggaaaacacaatccacaatctgaaagtagtctaggcaggctcatttttttgttgaaggaattcacatggaggcaattctgctcagttccagagagagattcttatcatcaaaagcacacacaataaccttgcttcaccacctgccactttctccagtggcctcttgttgtgaccagtaattgagaaatgacaaatgggtatagagccaaatctctaaaacagggacaccagtgtctcctagtatctgggtaataacctcctttcagtcttagtccacaccacacactaccctccagtctctcctactctttactgtcacagaaaagactctcagcttttattcacacctgccttcagaaggccaaaccattttgtgcctgaaaactgttacccactcgccccacactttacataagtatcacatatgttctttctacaaattggtatacaggtgccatttaatccattcaaatttggaagctacatcttcaagggtctgagagagctcactccccccatatattccccctttacatgttttcttataagacatacagtttaatcaattaacaaactaaacagcttatatactggcaatatattacagatgggtttatgtcagagtaatagatcacatgaaatggaccatgtggtaccccagtgcattatgtcttggtagagccctgaggacactgacagtagcatctctaagtaagtagtgctgtatgaatacagacacatgcggatctgtatctacatccatctgactaggccaaggagcaggtagatgcaagatagagacacacacatgctggatggggccactgcacaccttgtcatgccatttaaaagggcagttacaggttgccggttttgcagccattaaaattacactttatggaaaaggcttctctaattgtgtctgatttgctttctgtagtaagcatcattggaagaagaccaaagcaagagcaactagaagttaaatatacatttgagcttagctgcaatacagaaccctggggaagaagcaggctgaaagatttatttaattttaggcttggattctctcccttgctgttttcttgatgttgtgtgtctgcatttgtgtgtgtgtgtgtgtctgcgtgtgtgtgtgttccatcacatcatctcctgaagaacgctgggtttcgcaggcaggcggctagtcacctgcaacaacccaggggtcctgccgaggcttccaggctgctgtcagtgtcagatgccagggtctggtcggtggacatggaggagatgtcattgacagacgaggatggagggagactctcactgctgttcactgctgcacctgtgctgaaggagaaggctgtccttttactacaccatttttagtcttttcttctgaattcattacttccttgtagataagttctttccattcttcaattgtgtgttctctttcatccaactgcttgtcatatatctgaggtggaggcgcctccacttcggctgggtcataccagacgttgatgtagggatgctgtaaggcgtcgtccactgatattctttttgctgggtcaatcactagcatctttgacaacaagtccctggcttggctggctttgagtttattgtgctcggagtccgctgggaagagggaatctgggaagagtttggggaaggtgagtcccgcatacttgggccgattctccacatagtttcttactgtgggttgcaatttcttcatgaattctggacatggtgttcctagttgttcaattaccttattccactggtcaatatcgttctccttgtagcccatccccaggatgacctcaggggctctgtaataacgtgtcaccacatatggagtcatcatgaagcttgtgcctgctgtcctggccagtccaaagtccaggattttcaatgtgcaatcagacttgactacaatgttacttggttttaaatccctgtgaataattccagcagaatggaggtgcttaatgccacacaacatttggtacagcaggtaagacattcgctcatggtctaattccatctgaatcacttgacataagttggcatccatcagttccattactaagtaaacatcttggaactcctccagcgttttctggggtgtgaagacatttaataaactaataatgtttttatggttcacacacttcatgaggaccagctcccggtacgctctcttggcatgtgtttggttctgaaagggtctgctgagcttcttaatggccacatttctgtcaaggacagcatcatacgcggcacaaactatgccctgagccccagagccaataggctttagattctggtagcgcttgagaactgtgaaggttgagtctcccacttccacactgtagaactggttgtcaactttgcttttgctcatgttgtaatgtttggcaatatatgacacatccacttgtttatcgaatcccttgttttacctgtaaggaacacacacctgacaaaaggcaattttcacatccaatgttggttcactgcagtagtataagaaatggaggctcataaataccacagcttgtatggtttctcatctataggaaacgggtctaattcaacagtttcttgcataagttgccatagtgaagatctgagatgggcctgctgttggtgtttctcacactagccattccgtgcctgagaactacgatcctgatccggcagtgtttgccccagaaatcctccctacttgtttttcattaaccacattccagactaacatggaagagattctttggagatatggagattgtttaaaattaacgatggacaggtgatttccaagaaaacccaatcttaaactcactcaagcccctaggaattgaggggtgaggacaaaaaaggaaatttgtaaaaatgaaaaaagaaaagaaaaaggtaagcatatagcaagcaccacccacccccataaaaataaaaagtgaaggggaggttaaagaaaatagaagaagagtggcttgctgaatcaccctctttcactgcctggaaaccattgtgcagcgtgatgctgcctgtaccattgtg

SEQ ID NO: 9224 - RNA, 4440 nt, Homo sapiens
  source 1..4440: mol_type = other RNA
agacagtagttcttgcctggtttactctgagggggaaattcaccacttatgcaggtacgagagatagcctgtcaagcactttgaagatgctggctggagacttccttctgtcttgtgatgtcatcttgcggctgatgaaattccccttgagactctctttaaagcagcttcctgctctccgcacttaatcccatgtggtataaagtaagggaggggagaagccacagatatatcaagagaaaagtaccgagaaagaaaatcagtaaagaattagagatacagagaggagaagtttttaaaaaaaaaaaaaaaaaacaggaatatgaaagagagggagctcaagtgactgaggaggcatttttaacaatcaggttatctgcaatattaaccagaaaaaaaatggtagcaaaatagagaaaatgggccatttttattccaggggacaagctgcacaaaggaatgttcttctatttattttaaacaaatgactgcgtgtactgaatctgactgtgtgaaataatctcagaatggcagcaccactggcatggcgatggtgcaggtgggtgcagttccctgtggtctctattgcttgaagagagaaagaaagttccctattattatatttaaggcagttttcagagcactggcattcttgtttgctctgttttggggatattctatttgccaatcagttcacactcatcaaccatccacttcctgtctttcacttcttcaggtgaaatatcaccactctagtgagcaccaacatggtcagagtgcaaataactgtgatggatacttcgaagtgaataagaagggaagcctgattattgctgagatcaccttggtattgccttgtacataaccaagatgtttcacagtgcctccttaagtgctcaggaaagcactttcatttaatttaatttaagctaaattctggagattttgctaaacattgacattaatgcttcatggcttttaagacaaactcatattgctaaaactatttggcagcagtaaatttatgggcagagttattgctcttacatctactgcagtacaaaactcagatgatcagcccttcgattgctcatacttattaaaataaataaataaacatgaaacatcagccacattaaggagtcagggaaactcctgaggaataacaatgtctctggagatgttttcaaatgctaacctgagactcacactgtggtttgggggtttcattattattattattattttatttcagaagaggaaagtaatattatttctcaaaataaaactttggcagagtatgaatcagggaagcagcccacacatggaaaacacaatccacaatctgaaagtagtctaggcaggctcatttttttgttgaaggaattcacatggaggcaattctgctcagttccagagagagattcttatcatcaaaagcacacacaataaccttgcttcaccacctgccactttctccagtggcctcttgttgtgaccagtaattgagaaatgacaaatgggtatagagccaaatctctaaaacagggacaccagtgtctcctagtatctgggtaataacctcctttcagtcttagtccacaccacacactaccctccagtctctcctactctttactgtcacagaaaagactctcagcttttattcacacctgccttcagaaggccaaaccattttgtgcctgaaaactgttacccactcgccccacactttacataagtatcacatatgttctttctacaaattggtatacaggtgccatttaatccattcaaatttggaagctacatcttcaagggtctgagagagctcactccccccatatattccccctttacatgttttcttataagacatacagtttaatcaattaacaaactaaacagcttatatactggcaatatattacagatgggtttatgtcagagtaatagatcacatgaaatggaccatgtggtaccccagtgcattatgtcttggtagagccctgaggacactgacagtagcatctctaagtaagtagtgctgtatgaatacagacacatgcggatctgtatctacatccatctgactaggccaaggagcaggtagatgcaagatagagacacacacatgctggatggggccactgcacaccttgtcatgccatttaaaagggcagttacaggttgccggttttgcagccattaaaattacactttatggaaaaggcttctctaattgtgtctgatttgctttctgtagtaagcatcattggaagaagaccaaagcaagagcaactagaagttaaatatacatttgagcttagctgcaatacagaaccctggggaagaagcaggctgaaagatttatttaattttaggcttggattctctcccttgctgttttcttgatgttgtgtgtctgcatttgtgtgtgtgtgtgtgtctgcgtgtgtgtgtgttccatcacatcatctcctgaagaacgctgggtttcgcaggcaggcggctagtcacctgcaacaacccaggggtcctgccgaggcttccaggctgctgtcagtgtcagatgccagggtctggtcggtggacatggaggagatgtcattgacagacgaggatggagggagactctcactgctgttcactgctgcacctgtgctgaaggagaaggctgtccttttactacaccatttttagtcttttcttctgaattcattacttccttgtagataagttctttccattcttcaattgtgtgttctctttcatccaactgcttgtcatatatctgaggtggaggcgcctccacttcggctgggtcataccagacgttgatgtagggatgctgtaaggcgtcgtccactgatattctttttgctgggtcaatcactagcatctttgacaacaagtccctggcttggctggctttgagtttattgtgctcggagtccgctgggaagagggaatctgggaagagtttggggaaggtgagtcccgcatacttgggccgattctccacatagtttcttactgtgggttgcaatttcttcatgaattctggacatggtgttcctagttgttcaattaccttattccactggtcaatatgatcagtgccaggaaacagcactgcaccttttatcatttctcccatgatgcaccctactgaccacatgtcaacgttctccttgtagcccatccccaggatgacctcaggggctctgtaataacgtgtcaccacatatggagtcatcatgaagcttgtgcctgctgtcctggccagtccaaagtccaggattttcaatgtgcaatcagacttgactacaatgttacttggttttaaatccctgtgaataattccagcagaatggaggtgcttaatgccacacaacatttggtacagcaggtaagacattcgctcatggtctaattccatctgaatcacttgacataagttggcatccatcagttccattactaagtaaacatcttggaactcctccagcgttttctggggtgtgaagacatttaataaactaataatgtttttatggttcacacacttcatgaggaccagctcccggtacgctctcttggcatgtgtttggttctgaaagggtctgctgagcttcttaatggccacatttctgtcaaggacagcatcatacgcggcacaaactatgccctgagccccagagccaataggctttagattctggtagcgcttgagaactgtgaaggttgagtctcccacttccacactgtagaactggttgtcaactttgcttttgctcatgttgtaatgtttggcaatatatgacacatccacttgtttatcgaatccctgacaaaaggcaattttcacatccaatgttggttcactgcagtagtataagaaatggaggctcataaataccacagcttgtatggtttctcatctataggaaacgggtctaattcaacagtttcttgcataagttgccatagtgaagatctgagatgggcctgctgttggtgtttctcacactagccattccgtgcctgagaactacgatcctgatccggcagtgtttgccccagaaatcctccctacttgtttttcattaaccacattccagactaacatggaagagattctttggagatatggagattgtttaaaattaacgatggacaggtgatttccaagaaaacccaatcttaaactcactcaagcccctaggaattgaggggtgaggacaaaaaaggaaatttgtaaaaatgaaaaaagaaaagaaaaaggtaagcatatagcaagcaccacccacccccataaaaataaaaagtgaaggggaggttaaagaaaatagaagaagagtggcttgctgaatcaccctctttcactgcctggaaaccattgtgcagcgtgatgctgcctgtaccattgtggaacct

SEQ ID NO: 9225 - RNA, 4460 nt, Homo sapiens
  source 1..4460: mol_type = other RNA
agacagtagttcttgcctggtttactctgagggggaaattcaccacttatgcaggtacgagagatagcctgtcaagcactttgaagatgctggctggagacttccttctgtcttgtgatgtcatcttgcggctgatgaaattccccttgagactctctttaaagcagcttcctgctctccgcacttaatcccatgtggtataaagtaagggaggggagaagccacagatatatcaagagaaaagtaccgagaaagaaaatcagtaaagaattagagatacagagaggagaagtttttaaaaaaaaaaaaaaaaaacaggaatatgaaagagagggagctcaagtgactgaggaggcatttttaacaatcaggttatctgcaatattaaccagaaaaaaaatggtagcaaaatagagaaaatgggccatttttattccaggggacaagctgcacaaaggaatgttcttctatttattttaaacaaatgactgcgtgtactgaatctgactgtgtgaaataatctcagaatggcagcaccactggcatggcgatggtgcaggtgggtgcagttccctgtggtctctattgcttgaagagagaaagaaagttccctattattatatttaaggcagttttcagagcactggcattcttgtttgctctgttttggggatattctatttgccaatcagttcacactcatcaaccatccacttcctgtctttcacttcttcaggtgaaatatcaccactctagtgagcaccaacatggtcagagtgcaaataactgtgatggatacttcgaagtgaataagaagggaagcctgattattgctgagatcaccttggtattgccttgtacataaccaagatgtttcacagtgcctccttaagtgctcaggaaagcactttcatttaatttaatttaagctaaattctggagattttgctaaacattgacattaatgcttcatggcttttaagacaaactcatattgctaaaactatttggcagcagtaaatttatgggcagagttattgctcttacatctactgcagtacaaaactcagatgatcagcccttcgattgctcatacttattaaaataaataaataaacatgaaacatcagccacattaaggagtcagggaaactcctgaggaataacaatgtctctggagatgttttcaaatgctaacctgagactcacactgtggtttgggggtttcattattattattattattttatttcagaagaggaaagtaatattatttctcaaaataaaactttggcagagtatgaatcagggaagcagcccacacatggaaaacacaatccacaatctgaaagtagtctaggcaggctcatttttttgttgaaggaattcacatggaggcaattctgctcagttccagagagagattcttatcatcaaaagcacacacaataaccttgcttcaccacctgccactttctccagtggcctcttgttgtgaccagtaattgagaaatgacaaatgggtatagagccaaatctctaaaacagggacaccagtgtctcctagtatctgggtaataacctcctttcagtcttagtccacaccacacactaccctccagtctctcctactctttactgtcacagaaaagactctcagcttttattcacacctgccttcagaaggccaaaccattttgtgcctgaaaactgttacccactcgccccacactttacataagtatcacatatgttctttctacaaattggtatacaggtgccatttaatccattcaaatttggaagctacatcttcaagggtctgagagagctcactccccccatatattccccctttacatgttttcttataagacatacagtttaatcaattaacaaactaaacagcttatatactggcaatatattacagatgggtttatgtcagagtaatagatcacatgaaatggaccatgtggtaccccagtgcattatgtcttggtagagccctgaggacactgacagtagcatctctaagtaagtagtgctgtatgaatacagacacatgcggatctgtatctacatccatctgactaggccaaggagcaggtagatgcaagatagagacacacacatgctggatggggccactgcacaccttgtcatgccatttaaaagggcagttacaggttgccggttttgcagccattaaaattacactttatggaaaaggcttctctaattgtgtctgatttgctttctgtagtaagcatcattggaagaagaccaaagcaagagcaactagaagttaaatatacatttgagcttagctgcaatacagaaccctggggaagaagcaggctgaaagatttatttaattttaggcttggattctctcccttgctgttttcttgatgttgtgtgtctgcatttgtgtgtgtgtgtgtgtctgcgtgtgtgtgtgttccatcacatcatctcctgaagaacgctgggtttcgcaggcaggcggctagtcacctgcaacaacccaggggtcctgccgaggcttccaggctgctgtcagtgtcagatgccagggtctggtcggtggacatggaggagatgtcattgacagacgaggatggagggagactctcactgctgttcactgctgcacctgtgctgaaggagaaggctgtccttttactacaccatttttagtcttttcttctgaattcattacttccttgtagataagttctttccattcttcaattgtgtgttctctttcatccaactgcttgtcatatatctgaggtggaggcgcctccacttcggctgggtcataccagacgttgatgtagggatgctgtaaggcgtcgtccactgatattctttttgctgggtcaatcactagcatctttgacaacaagtccctggcttggctggctttgagtttattgtgctcggagtccgctgggaagagggaatctgggaagagtttggggaaggtgagtcccgcatacttgggccgattctccacatagtttcttactgtgggttgcaatttcttcatgaattctggacatggtgttcctagttgttcaattaccttattccactggtcaatatgatcagtgccaggaaacagcactgcaccttttatcatttctcccatgatgcaccctactgaccacatgtcaacgttctccttgtagcccatccccaggatgacctcaggggctctgtaataacgtgtcaccacatatggagtcatcatgaagcttgtgcctgctgtcctggccagtccaaagtccaggattttcaatgtgcaatcagacttgactacaatgttacttggttttaaatccctgtgaataattccagcagaatggaggtgcttaatgccacacaacatttggtacagcaggtaagacattcgctcatggtctaattccatctgaatcacttgacataagttggcatccatcagttccattactaagtaaacatcttggaactcctccagcgttttctggggtgtgaagacatttaataaactaataatgtttttatggttcacacacttcatgaggaccagctcccggtacgctctcttggcatgtgtttggttctgaaagggtctgctgagcttcttaatggccacatttctgtcaaggacagcatcatacgcggcacaaactatgccctgagccccagagccaataggctttagattctggtagcgcttgagaactgtgaaggttgagtctcccacttccacactgtagaactggttgtcaactttgcttttgctcatgttgtaatgtttggcaatatatgacacatccacttgtttatcgaatcccttgttttacctgtaaggaacacacacctgacaaaaggcaattttcacatccaatgttggttcactgcagtagtataagaaatggaggctcataaataccacagcttgtatggtttctcatctataggaaacgggtctaattcaacagtttcttgcataagttgccatagtgaagatctgagatgggcctgctgttggtgtttctcacactagccattccgtgcctgagaactacgatcctgatccggcagtgtttgccccagaaatcctccctacttgtttttcattaaccacattccagactaacatggaagagattctttggagatatggagattgtttaaaattaacgatggacaggtgatttccaagaaaacccaatcttaaactcactcaagcccctaggaattgaggggtgaggacaaaaaaggaaatttgtaaaaatgaaaaaagaaaagaaaaaggtaagcatatagcaagcaccacccacccccataaaaataaaaagtgaaggggaggttaaagaaaatagaagaagagtggcttgctgaatcaccctctttcactgcctggaaaccattgtgcagcgtgatgctgcctgtaccattgt

SEQ ID NO: 9226 - RNA, 44 nt, Homo sapiens
  source 1..44: mol_type = other RNA
agacatcaagatcagtcccaaatatttcagtttattataaacaa

SEQ ID NO: 9227 - RNA, 43 nt, Homo sapiens
  source 1..43: mol_type = other RNA
agacatcaagatcagtcccaaatatttcagtttattatagaca

SEQ ID NO: 9228 - RNA, 12699 nt, Homo sapiens
  source 1..12699: mol_type = other RNA
agaccctgcagccttcccacccttccccaggccgctctccccagccctggcctcctgcgttcctcttgtgcagcttctctcgggcacagacacaaacctcaccggagttgtgtgggaagatcccaaagcccttcccaatgccaccctgcagggtactgggatgcatgggggtagttgtggcctgtggtcccactcatgcccctgcttcttgtccctcatgtcacttctttcccaggtgaacatggtccttttttgccttcagtccccaaatccacctgtacaaatttgccagatatggcaggctctccatgaaggttttgggataacacagagggagcacagcgtacccaccaaacagaacaaccttgaggtagaatagggtctgaaggcagggaacctaaggctgtttcacattgacttcatagaactaaattgaaaggaaaaccctaactttccatgcctaagtaacaaaaggaccagaggctactccctttgcaaacccccaccttttctacagggcagatgggaaactgaaagtatctctgattggtgccaagcaaccaatcagatgtttgcataggagtgtaacttcataacttcacttcagcctctgactggttgctgtccacagccaatcagactgattgcggaccaagtcttcctttgcataaaagtgcaactttgtaacttcaccttagcctctcatgctaaagtgaatcttaggagtttgcataggagtgtgacccttgtaaccacttcagcctctgagtggaaagcaaccagattgattgcaggccaccacttcatttacatgggtgaacaccaggtggccagtgggaaacctctaggaggtatttggacccaagaagattgtgtatcaggacccttgtgtccctatgctcgggcccacccccacactgtggacagtactttcattttcaataaatctctgcttttgttgcctcactcttcccttactttgtttgtgtgttttgcccaattctttgttcaagatgccaagaacctggacatgcttcaccaacagcaacctgaaattgaaaaccgctaatcattgttcttaaaaggtccttggccatccaagccctgggggttttctactggcagccctgatctcatactcatcccaccaccagtccctgggtcctccccatccttctgctcttatctccactgcttctcctttcccaggctcttcttccctctccagagctaccctgacatttcagtttcatcttcttttattgtactgtgtgtttcagcaatctgagtgttactgtctcccactcatcctcaccttttgaagaaagaaccaaaaacaaaaacaaaaaaagtcaatataggcctttcaagatactccaaaaacttaagaaaaaagtgttaaggctatattacaagaccccagaaaaatgatgctcagaagacaaaagcagtaatttttagtttaaatagtactttttctctggcagtaagtacatcagggagagtcaagacttcctcttggaaaagtatgccatctggttcttgtcatactgttgtgctccttaactcatttcatgcaaaatttccagcaccatgtttgagggaccctgattactcctcatccatgcagtttcagagccacaggagagatgcatgtgggtgggcagaagtggaagttgtttatgagcatgaagtatttctgagaaatgaacgcattgatgttgggatttgaaatctgatttatctctttgatgattacgggaggaaattttattataaacaataatatttgctggcatatgcatggatgtctgaactcagatgataaaaactagaggattttgagcatcttggaaaaaaattgtacaattaatttaagatttcttacatgacctagaaaatgaaaaggggaagcaaatacactggaaaaaaaagaaggtggaggaggatcacattactccttcacagttaattagaagaactttcaaccaaaacacataactgggtaacaaataccaggtaattttctttgactgaattttttttcacttcattttctttgaagtgaaaaaaagtaatttttaaatacaggaaataatattttatgactgagtattctcttcaaagaatctgggtcagcagctcatttcaaattttcagtgcctagaggacgataatacttagtgctgtttgctggtgatttacaacactttcgtggcttaagaccaagaatatacatattaaaaatcatgctctgcctgaatccaacaagcagatgccccaccttcttttaaggaagaacatgacaataatgaacggataatagagtacaaacaaagacactcaaactgcatttcctaatgttgcaaatgttaatattgagtaacaaagcatcatttctattaaagctggccttcagccactcccttatgaggtaggtggaaagaaatctttttactttcccataattctactacttacgggaaagcaagttgactttgcccagcattgatgcaaagagcatgacacagagttcaagccgcagcactgctgctcaggagagtggaaaagagaaaagttattggcacaatagcaaccaagtgtttcatctaaatgttctgtttcttgagctcccaggtaactcagcttcacatcttttccttgtacaggtcaactccacttaggtagaatgtgaatatatagtatgagaggccaaaaacccatacctatataagcaaaattatctccccctactgccaattcataaaaataacacctgccagaatggaacagaatgctgaaaagtctaccttgaaaagatgagcgattttcaagccaagaaaacttgaatgtatgaaaccccctagaaagaatgtgtcatccagggggtaattggcccatcgcagaaacatggaaaagaggaaaaggaagacagcagggcacagtgttcataagaaagagacacaggatgctttttaagaaacttgggtgtgaaagcaaaacaggcaatatttagaaaggaacttttggtcaatgggtggaaatgggttaaaataggagccatttgcacataattatattctaaggggaaggaagcaatagagagagcaattgaaaatgtaaggaagagagggaagaactgatgtgggtgagggtgcatgtttagaacacaggctgggaagagtcggccgcgggagtcacactgctaataaaaggcagagaccaggggtttttggacctgggtgcaaattgtggtcttgccactttctatctgagggaccttgtcaccctgatggtgaaaaacaagcctgtaacagaagaaaggaaagacaagaactgggaggctgtgataagggagctgcatatatcagcagtgcagcaagtctggctgttgacatggttcttggtgagcccaagagagctgactgctggaaaagagtagaggagaacattttcagcctcagaaatatcactggcctctgatgggagagataagtggtctcagggcctaatgagtgctggagaattcattcattcattcagtgaacatgactgaggcctctcactttgctagacattttggaagacaggggtcaaaatcacagttcctactctcaattagctcacagccctgtactagtgatggacaaagaaccagtatgtgacagttcagactaataagcccaacaagagagggatatacaggacactgtgggacccctaaagggagcaccttgtgcagaggtagaaggataggaatgaacgaggggtgacgggtaacaggaagagagagaagcaccgcaggagtctctgaagagtgttcacagggggtgcgaggcttgctgtgcagaaaccaataggggcaggtgagaaatgctgaccccaagggatgagcaggctcatgtcagggtgctacaaccgtcccctcctcttcactctttcctgcaccccagactccaagtcttaaactaggttatctccccagtggcctggcctgccccccgaatgctctcaaaccagtatcttctaaccctagtcaaaaattaccccttcccttcagctagccattagaattgaaacaaattcccactgccatgtgaaagtctgattatcctactgttcccaaggcaccagccttttagtgggatgtttgctgtagtagattgtatcttccaaaaatggccacaaaatgtttctgagtccacatgctcatccagaaactttctactccctcattaagagatagaatctatttcccttccccttgaaattgggctgcctttgtgacttcttcaataaaaagagctgcttggaacccccacccacagcccttacctcccctgcatccatgagcacacccctctgggactatactgtctaccattgcctccctgacttgggactttggctctggagttcactccctaccccaaggccataaaaaacccccactgcactctttagtccctgggctccagccactgccctctccccagatttctctgttttctgccatctctgtgggatccgcataatctgcctccagcagtttctgggagtgaacccagctatcttgctgaaggtagggtaggggtggatgcaacaatgggctgattgttatcaatatgtatggcaagatattatcttgagatattaatctgtgggtttttctttgctcacttccttgtacagtgaccaaacagcctcacgcaagagtacagttggtaaagagggactgaaaagagccaaaaatgtcaacgttcatatttgtgactctaaaacagcatccaagaatcaaaaaagcaaggcttggggcacaaagcacagagacatgtggaccagggacagggatatacagacagccctatcccagtgcctccagggagaccagagtaaggtgtgctgggccgagggaggggaggagcacatggtgaggagcaggtccacattggaagtcttgggagccccaggagcccctcagctggttgcatattcccagagatgtttgccaagccctgattacatatccacactcccctgaatgaacacaccctccccattccagtgtctaaggactctcatgagccctgcagatctgttaggaacactttcagctctaagcaacaaaagatatgattaacagtgccttaaacactacaggtgtattctttcacacaacaagaaggctgtaagtgggtagtttgttggtaaaaatgcagtttatccaggacctagctcatgagcttaggattcaactagttctggaatcatccttaggaatctataattctgaaaacttcctaggtgattctaatttgcaatcagatatggaagccacttctcccaagtttactaaggctgctgtactctcccctcttctgagttttcggagtccattagctttcagaggagtcaacagtgctaccagtgaacacctgactaatttattcactcaaatggtcagcacaccgtaattgctcgctttttacctggtagcatcagctcagtgagggttgtgaactgggcctagagacatgagaattcagcagcatttccaaactgggtagaatttccacagactatttcaagtgctttttttttttccattcaagaaagatggggcaaccagccaagtaaacatggttgtttttgtctgttttgtgttgctaaaacagaatacctgagactgggtaatttataaacgatgatttatttggctcatgttctggaggctggtgctggaatctggtgagggccttctggctatgccattttctggggaaacatgtggaactttcaactagccgcgccagttgaaaatgggactggtttctctgatgagaatggctgggtaggaaatggtaatctgtcagaccacaaggaatttttctagtcaacaaactccagatgtttgtgattcttttcctcctggttcactgggttcagccaaagtcctccctagaagattgccaagtgtaagctgagcttgaatctgttccgtgctcccttcttactgatacaacctcgaccagttacttaattctctgtggcacccagtttagtcctcaaacttgtggagattaaacaagattattctcggatcacacaggtcaagcagggctataaaaccgggcagcctggctccaagtctactctctgagccactgtgcaacctacaaacgataacagaaaagaacccaaagacttaacagttagagaaagcccctctgaccccaagcattctctctgttcccctaaccattgttagtcatttctgatttgtccttccagagacagtctgtgtgcacatctttctaaatgcacatctagaaagaagaagcttctgatatcaccttgggcagtcacactcatgcacaaataggagatgtttttatcttttctaataactgatatcaactttgctttccaagtccctatttgggtgcttacactggtgagtgcaggggcaaggacagaggagaaaatagtctcaacgaagggtacctttgcaaaatactccatccaccccagtgtttctgctgtcttctctgatgtgactctcagccatgatgtaggttaaagcgtctatcttagggattccttctccttccccagggtcttttttcctctctccccacaaccctgctctccctcacagccttagagagggcagcagggcttgtggagctcagagacgatgctcaaatgggaacagacaattgtccagcgtggaagcagtcacttctgacctggggtcatggcttggcctggcccctgtggctgacaaggcactactgccatggctgggagttgctggtgaaaggaaatgtcccttctccagctgggtcatcccaaaattggtggactctgaagatatggtagtcccagtgcaggtagcagctgtggtgttcccagattgtttggcttccaccacacccggcactatctccccactgcctcccacctcccacccccagtacgaggcagccttagatctctgtgtttcctgccaatactaactgcctgttggatgaaaatccattaggaattttcaaccaacgttacaaaaccacactcaggctggctttaaccatgaaatagacttactggttctgagtctagagacagggcaggcttcagatgggtcacggtccagtgggttagtaacacccccaagggcctggtttctttccaggcttcatctctgccttccactgagtcgacaccatcctgagcctctttcctgagggaggcaagatggcaccaccagcttctggggcacacacttcctctcacatgcacggtagaggaagggagagcacacactctcagaagagcaagacaacttccctccaagactccaccaaccgcttctcctgacttacttgcccaaatagggtcctgagcctatccctgaacccaccacagtgacactgtctctctccagtcagattgccagaatgaggtgtgttcagcagcactggagagaggtgagcaaaggtgaaaatcagagcagcattagcaggaagaggggacagctgctgggaggccccccgcacacctgcgtccacatgccctcacctgttcttgatgtattctcagggcttggctaagagaacctggggcctgagatgcttgggaactggctcctgggccttcttacattccacaagctggggtggccaaaggtaaccaggatggcagtgtcactatgaccttctttctccgcagccaaccacctggtctcctcatgcccagtcctctcatctgctgcgaagacacatcccaggccctctgggacgggtttgctatagactgaattgtgtccccccagttcatgtgttgaagccctaacctccaatgtgatggtatttggaggtggggcctttgggaggcgattacagttagatgaagtctaaccataattactaatcccatgatgggattagtgtccttataagaagagacacagaggcttgccgcttccctctctgctgtgtgagcatgcagtttcaggccacgtcaggaagaggggcctcggcaggaactgaatcagccagcatcttgatcttggacttcccagcttccaatccatcgaaaacacatttctgttgtttaagccacccagtttgtggtattttgttatggcagaacaagttggttaagacaaggaaaataaacagccaatgcctctcagagccctctctctctgctctctggcctctttatgtagtcaagaggataggaggggggcaagtacagctgttcaggggctgctggatacgtctacctagcatagggcacagaagccaatgctgcaatctgctcagtcagaacttaggtctcttggctcaagacctggtccctatttaaataacagtacttccaagatgagcaatgcagtgagccgtggcagccactgacactacagtacgaatctgctcagcagctccttccctggaagtttcagtgtgaggaaacatgactaggtccgaggcaagaaagagtgtggcgaggcaagactcagagaaagggagacaagctggaactacacaacaagcaagcaaggcaggcaggctctggctacgcagaacgacagcactgtaaagctcctgtggcggtcttccctaccggaggagaaactgattgaagcgcattcggaaacagcacctcatttatttacttatttagaatagacaatatacattatacacacatgaaaaaagcaaccaccacaaaagagagccaatggtgaagagtttctctctcatcctatattggcaattcttataaacctttgcagagacagtttttgcatatttccacatttatgtatgttatttttttctttttaaacaaatagcagcatactacttgccctactctacaccttgctgttaacaacattataccttagagatggttcagtatcacacacacctcaatctacctcttcttcatgactgtacaatattccattctatggaggtactataattagtcaaccatgaaacacaggtgttttcccagcccttaactcttcattgtttaaaaaaaaaaatctgtattcgtgtctattgtgtgccagtcactgttctagggaatagagagtagaaaatgagacattcagtgtcactgccgtggaggagtttacaatccatatgtggaaatgaacatccttgcacatacttctttatgtacatgtgtgaatgtattgttattataaactctcaaggtggaattgctgggtcagagccatgtgcatttctaatttcaatagatattgcaaattgtccaccaaacaggtcatgtcagtttcccctctcaccgtctgtactatcttttcatatgattaaaagtcattatagctttatataccattaggtttcttaaacacaaagtaagttctctaaaatgctcatgataacctgagcaatgactaaggaactagggaacatgacatatcaggacacccttgtggggacacatctgcttctgtgcagaggctggggcagaacctgctggctgatactttcctcacctcctatgtggcacagtcttccagcagccctgggccaggggtgggatatgatgacaggtcttttggagaacgtggtggacagttagcaatgtcactcccccacacagtatgtggcaaggaagaagaatctgtgtacacacaaaatctgtctatgaactgagaaaaaacacagggatacccatgacagaccaaggcctgatttccctcgtattgaaagagcttctacaaatcaaccagaaatccaaccaccccacaggtaagtggacaaagaatatggacagttcttgcaaaggaaatactctgtgttccagaaaatccctgtttataaaataaatactataattaaatgtctacatgcattgctgatcagcatcaatttgcccccattgtaactgttatcactatttaaaatagctaacctcggaagagtgccctgagctcacacagcagcacttggtctcctggtcttttctgtcttccctcttgcttatgactttccatgattctcaccatctcatctcataggcaggaactgcacacacgctgcacaggctgcctgttggccactatcagccattcccacccttcccctcctcgcctcagtgacagaggtggctacttccttcccactaggcattatccctgcagggaccccactggggctctgcagattcccagatccctttctctgagtctgccccttccacttggcatgcttttgcttctgacctaaggctcctgcagctcttctgggagggctgttcttgtgctactgcccttttgtgcccacctatagaaagactgaagtacctgggttatcaacgagggtggctcttagccagtggctgacaggcatagaagaatggaagcccagataccctgcctggggcagggacatctcagaggcattgtttacagttgagagctccccttcaggtcaggctgaacctacctgtcatataactgtctgagatccttgcatggctatccttcttctagctccttactgaattctgctcggagcatttcttttaggaacaatctttgtttctgggcctgcttctaggaaacccaacgtaagacacaatcttcttcctcagtaacaaaatcctgagttttattttggcatatggccaccgtgaataaaaactacatttcccagcttcctttgcaaccaagttcttgccaataagatacagggcacaagtgccctgtgagacttctaggaaatccataaagggagtcctgctgatggctagtgtccatcgtggaccctgagggcaaggggtacatcctcaggatgtgggagcagagatctggaaaaggcctggacctctaacaacctcatggatctgccaataccaaccgcagattgtctaccatcccaccattaccccacaacttcttttgagaaataagttcctctcctgtttaagccaatgtcattcgggtgtttattccatgcagttaaatttaatcctagtttacagaccagaccattgactctgaaaaacgacagacactcagtttgccagcctcccttgcagctaggctttgccagtgtaacccagatctggctgaggaggtataaaggaaggtcttggggggaagaaaggtgtaggcaggaggttctggaaaagatatttcttcctgatgcaaaaaacaaacaggtgcacaatgtccagctctctttccactctggcaacctattccctgctacctgcctttggctgcagcatgtgaagatgtgctgtctggagctgtggcagccattctataaccaggaaactacaagtgcatggacaaaaagccaaccagctgaggatggctgtgcagaaggatggagagagcctgggtctttcagaaactcactgagatctcccactccaaaccaataaatggtccacactgttaatcgggttttccattacatacagttgaaagcaatctaacatactcacagggaacaaagcactgaagtaaaatcacctggaagtgatcaattctcaaaaagcctgctactataacctcttggagggtgctatagtttgggtgtttttgtcccctccaaaattcatgttgaaactcaattcccagtgcaagaatgttgggaggtggggcctagagtgaggtgtttaggtcataagagtgggtactctctcactcttccagcatgtgaggacacagcgttcctccccttcataggatgaagcacgcaaagccccattttggaagcagagacagagctaagaccccaccagacaccaagcctgttggtgcctggatcttggacttccaacctccagaactgtgagaaacagatatctgttctttataaattacccagtctcaggtattctattattgcagcacaaaacaaactatggggagatgactgggttctgggaggtgattacctgtgctaggcttgcctctgagggcaagaaacagcaactccagcttcagggaagtgaaataataagaaataaactccaggatccgctgattcctgtgttcaacaatgccatcaggaacccagggccctcccctctctctgctctgccactcttgaaatgggcttcattctcaggcagccagcaagacagaggcatgcttctgggcagcacagccagacctaactggggcctatcgagggcctgcactctcccccttggcttctccctccagctggattttcttgcttttcttcaaacatgccagataggctcctgccctagcctctgcacttgcgttccctctgcctacagtgcttttgcatacatgtccacttggctctgcctccttcaggtcctcacccaaatattacctcccgagagaggcctgccctgaccacaccttttaagattaaccacctcccaactccccatttctttttctggcttaatttttctccctggcatgtaacttcatccaatatagcacacattcccttggcctcactgagtgtccgggccccacttgcctagaaggtgtgctccaggaaggcagagatgtttaagattgttcaccctcattcccccagggcctggcacaggtgtttcacaattatcttcgccctgggggcggaggggaggggcccaccacggccttatttccgcgagcgccggcactgcccgctccgagcccgtgtctgtcgg

SEQ ID NO: 9229 - RNA, 11924 nt, Homo sapiens
  source 1..11924: mol_type = other RNA
agaccctgcagccttcccacccttccccaggccgctctccccagccctggcctcctgcgttcctcttgtgcagcttctctcgggcacagacacaaacctcaccggagttgtgtgggaagatcccaaagcccttcccaatgccaccctgcagggtactgggatgcatgggggtagttgtggcctgtggtcccactcatgcccctgcttcttgtccctcatgtcacttctttcccaggtgaacatggtccttttttgccttcagtccccaaatccacctgtacaaatttgccagatatggcaggctctccatgaaggttttgggataacacagagggagcacagcgtacccaccaaacagaacaaccttgaggtagaatagggtctgaaggcagggaacctaaggctgtttcacattgacttcatagaactaaattgaaaggaaaaccctaactttccatgcctaagtaacaaaaggaccagaggctactccctttgcaaacccccaccttttctacagggcagatgggaaactgaaagtatctctgattggtgccaagcaaccaatcagatgtttgcataggagtgtaacttcataacttcacttcagcctctgactggttgctgtccacagccaatcagactgattgcggaccaagtcttcctttgcataaaagtgcaactttgtaacttcaccttagcctctcatgctaaagtgaatcttaggagtttgcataggagtgtgacccttgtaaccacttcagcctctgagtggaaagcaaccagattgattgcaggccaccacttcatttacatgggtgaacaccaggtggccagtgggaaacctctaggaggtatttggacccaagaagattgtgtatcaggacccttgtgtccctatgctcgggcccacccccacactgtggacagtactttcattttcaataaatctctgcttttgttgcctcactcttcccttactttgtttgtgtgttttgcccaattctttgttcaagatgccaagaacctggacatgcttcaccaacagcaacctgaaattgaaaaccgctaatcattgttcttaaaaggtccttggccatccaagccctgggggttttctactggcagccctgatctcatactcatcccaccaccagtccctgggtcctccccatccttctgctcttatctccactgcttctcctttcccaggctcttcttccctctccagagctaccctgacatttcagtttcatcttcttttattgtactgtgtgtttcagcaatctgagtgttactgtctcccactcatcctcaccttttgaagaaagaaccaaaaacaaaaacaaaaaaagtcaatataggcctttcaagatactccaaaaacttaagaaaaaagtgttaaggctatattacaagaccccagaaaaatgatgctcagaagacaaaagcagtaatttttagtttaaatagtactttttctctggcagtaagtacatcagggagagtcaagacttcctcttggaaaagtatgccatctggttcttgtcatactgttgtgctccttaactcatttcatgcaaaatttccagcaccatgtttgagggaccctgattactcctcatccatgcagtttcagagccacaggagagatgcatgtgggtgggcagaagtggaagttgtttatgagcatgaagtatttctgagaaatgaacgcattgatgttgggatttgaaatctgatttatctctttgatgattacgggaggaaattttattataaacaataatatttgctggcatatgcatggatgtctgaactcagatgataaaaactagaggattttgagcatcttggaaaaaaattgtacaattaatttaagatttcttacatgacctagaaaatgaaaaggggaagcaaatacactggaaaaaaaagaaggtggaggaggatcacattactccttcacagttaattagaagaactttcaaccaaaacacataactgggtaacaaataccaggtaattttctttgactgaattttttttcacttcattttctttgaagtgaaaaaaagtaatttttaaatacaggaaataatattttatgactgagtattctcttcaaagaatctgggtcagcagctcatttcaaattttcagtgcctagaggacgataatacttagtgctgtttgctggtgatttacaacactttcgtggcttaagaccaagaatatacatattaaaaatcatgctctgcctgaatccaacaagcagatgccccaccttcttttaaggaagaacatgacaataatgaacggataatagagtacaaacaaagacactcaaactgcatttcctaatgttgcaaatgttaatattgagtaacaaagcatcatttctattaaagctggccttcagccactcccttatgaggtaggtggaaagaaatctttttactttcccataattctactacttacgggaaagcaagttgactttgcccagcattgatgcaaagagcatgacacagagttcaagccgcagcactgctgctcaggagagtggaaaagagaaaagttattggcacaatagcaaccaagtgtttcatctaaatgttctgtttcttgagctcccaggtaactcagcttcacatcttttccttgtacaggtcaactccacttaggtagaatgtgaatatatagtatgagaggccaaaaacccatacctatataagcaaaattatctccccctactgccaattcataaaaataacacctgccagaatggaacagaatgctgaaaagtctaccttgaaaagatgagcgattttcaagccaagaaaacttgaatgtatgaaaccccctagaaagaatgtgtcatccagggggtaattggcccatcgcagaaacatggaaaagaggaaaaggaagacagcagggcacagtgttcataagaaagagacacaggatgctttttaagaaacttgggtgtgaaagcaaaacaggcaatatttagaaaggaacttttggtcaatgggtggaaatgggttaaaataggagccatttgcacataattatattctaaggggaaggaagcaatagagagagcaattgaaaatgtaaggaagagagggaagaactgatgtgggtgagggtgcatgtttagaacacaggctgggaagagtcggccgcgggagtcacactgctaataaaaggcagagaccaggggtttttggacctgggtgcaaattgtggtcttgccactttctatctgagggaccttgtcaccctgatggtgaaaaacaagcctgtaacagaagaaaggaaagacaagaactgggaggctgtgataagggagctgcatatatcagcagtgcagcaagtctggctgttgacatggttcttggtgagcccaagagagctgactgctggaaaagagtagaggagaacattttcagcctcagaaatatcactggcctctgatgggagagataagtggtctcagggcctaatgagtgctggagaattcattcattcattcagtgaacatgactgaggcctctcactttgctagacattttggaagacaggggtcaaaatcacagttcctactctcaattagctcacagccctgtactagtgatggacaaagaaccagtatgtgacagttcagactaataagcccaacaagagagggatatacaggacactgtgggacccctaaagggagcaccttgtgcagaggtagaaggataggaatgaacgaggggtgacgggtaacaggaagagagagaagcaccgcaggagtctctgaagagtgttcacagggggtgcgaggcttgctgtgcagaaaccaataggggcaggtgagaaatgctgaccccaagggatgagcaggctcatgtcagggtgctacaaccgtcccctcctcttcactctttcctgcaccccagactccaagtcttaaactaggttatctccccagtggcctggcctgccccccgaatgctctcaaaccagtatcttctaaccctagtcaaaaattaccccttcccttcagctagccattagaattgaaacaaattcccactgccatgtgaaagtctgattatcctactgttcccaaggcaccagccttttagtgggatgtttgctgtagtagattgtatcttccaaaaatggccacaaaatgtttctgagtccacatgctcatccagaaactttctactccctcattaagagatagaatctatttcccttccccttgaaattgggctgcctttgtgacttcttcaataaaaagagctgcttggaacccccacccacagcccttacctcccctgcatccatgagcacacccctctgggactatactgtctaccattgcctccctgacttgggactttggctctggagttcactccctaccccaaggccataaaaaacccccactgcactctttagtccctgggctccagccactgccctctccccagatttctctgttttctgccatctctgtgggatccgcataatctgcctccagcagtttctgggagtgaacccagctatcttgctgaaggtagggtaggggtggatgcaacaatgggctgattgttatcaatatgtatggcaagatattatcttgagatattaatctgtgggtttttctttgctcacttccttgtacagtgaccaaacagcctcacgcaagagtacagttggtaaagagggactgaaaagagccaaaaatgtcaacgttcatatttgtgactctaaaacagcatccaagaatcaaaaaagcaaggcttggggcacaaagcacagagacatgtggaccagggacagggatatacagacagccctatcccagtgcctccagggagaccagagtaaggtgtgctgggccgagggaggggaggagcacatggtgaggagcaggtccacattggaagtcttgggagccccaggagcccctcagctggttgcatattcccagagatgtttgccaagccctgattacatatccacactcccctgaatgaacacaccctccccattccagtgtctaaggactctcatgagccctgcagatctgttaggaacactttcagctctaagcaacaaaagatatgattaacagtgccttaaacactacaggtgtattctttcacacaacaagaaggctgtaagtgggtagtttgttggtaaaaatgcagtttatccaggacctagctcatgagcttaggattcaactagttctggaatcatccttaggaatctataattctgaaaacttcctaggtgattctaatttgcaatcagatatggaagccacttctcccaagtttactaaggctgctgtactctcccctcttctgagttttcggagtccattagctttcagaggagtcaacagtgctaccagtgaacacctgactaatttattcactcaaatggtcagcacaccgtaattgctcgctttttacctggtagcatcagctcagtgagggttgtgaactgggcctagagacatgagaattcagcagcatttccaaactgggtagaatttccacagactatttcaagtgctttttttttttccattcaagaaagatggggcaaccagccaagtaaacatggttgtttttgtctgttttgtgttgctaaaacagaatacctgagactgggtaatttataaacgatgatttatttggctcatgttctggaggctggtgctggaatctggtgagggccttctggctatgccattttctggtggaagcgaaagagagagaaaacagggccaaactcatccttttatcaggaacccactcccacagtaactaacccactcccaagataatggcattaagactgtcctgatgacctcatcacctcttaaaggtcccacctgtcaacactgctgcattgaggattaagtttccaacacatgaaacttgagggacacatttaaaccataacaatggtgggctgaacattgtcttttgcctatattcccacccccaaaattcactacagtatcgagattttgttaaaggcaaaaaacaaataaacaaaccatctcaaggacaaggctaaaagagaaaggagcaagtgtggagagagagaggtaaacacgatgtcggaaaccggaaagcaggtggtaaatgatgagtaacttagagaccaggcacaggttgcagagaggaggcaggaagacaacagactggccccggagcacctggtaggcatagaattggaggccccaggaacctctctggttgtggggtgttggttaaaaggctatactaaatacagcttgatcctttgatcgcttctccactcccatcagacaaggcacctctctcatcctacagaagacataccagagaaggggataagggccaagtcagcatgctgaatggcgagaacagcctgcagcctttcgccactgcatctgagaatcctggtgactcagcttagacacatggggcgacaggctacaaatttcttctctggagaaactgagctcctcaaagaaaagacttataaacaatgactactggggattataatcaaatatacatattcagagaaagccaacacagcacaaaaagcagaataaactttaaggaaaactgtaattaatatcttcggagaaagaatataactgcatctacaaaaaagaacaaactactcataaaacaaaaatgagctctcagttctaaaaaaatataaaaacaggaaaaaaaaatccaatagaatccaaacaggctttactgggaaggtactggaggatatattccacaaaatgaaagagcaaaccaggaaaaaggcatacaaaggattcaagagagagggatccaactaaggagaactgaacgacacatcagagcaggaagccaatgggctccagaggggatgtgttaaaaataaaaaatcagttgattacctgatgtgtttgaactattaagaggagattaacactgctggcaatgcgttggaggagaattagggacagaaaaatatcaaaacaagataattttgaactccagggagaaaaagaagttgtataacaacggaagtattatcagtgtacactgtgtgccttaccggggaaaacatttataataatcacaacagttaactttgagtagttacttaattaaaaaatacaatataattacattggaagaataggggaacaaaagtgctcaatcttcatctttcataggaagaagtcaaagtttctgcctaatctgaaaaatcaacacagaagcatataatttagatacctggggaaacatgtggaactttcaactagccgcgccagttgaaaatgggactggtttctctgatgagaatggctgggtaggaaatggtaatctgtcagaccacaaggaatttttctagtcaacaaactccagatgtttgtgattcttttcctcctggttcactgggttcagccaaagtcctccctagaagattgccaagtgtaagctgagcttgaatctgttccgtgctcccttcttactgatacaacctcgaccagttacttaattctctgtggcacccagtttagtcctcaaacttgtggagattaaacaagattattctcggatcacacaggtcaagcagggctataaaaccgggcagcctggctccaagtctactctctgagccactgtgcaacctacaaacgataacagaaaagaacccaaagacttaacagttagagaaagcccctctgaccccaagcattctctctgttcccctaaccattgttagtcatttctgatttgtccttccagagacagtctgtgtgcacatctttctaaatgcacatctagaaagaagaagcttctgatatcaccttgggcagtcacactcatgcacaaataggagatgtttttatcttttctaataactgatatcaactttgctttccaagtccctatttgggtgcttacactggtgagtgcaggggcaaggacagaggagaaaatagtctcaacgaagggtacctttgcaaaatactccatccaccccagtgtttctgctgtcttctctgatgtgactctcagccatgatgtaggttaaagcgtctatcttagggattccttctccttccccagggtcttttttcctctctccccacaaccctgctctccctcacagccttagagagggcagcagggcttgtggagctcagagacgatgctcaaatgggaacagacaattgtccagcgtggaagcagtcacttctgacctggggtcatggcttggcctggcccctgtggctgacaaggcactactgccatggctgggagttgctggtgaaaggaaatgtcccttctccagctgggtcatcccaaaattggtggactctgaagatatggtagtcccagtgcaggtagcagctgtggtgttcccagattgtttggcttccaccacacccggcactatctccccactgcctcccacctcccacccccagtacgaggcagccttagatctctgtgtttcctgccaatactaactgcctgttggatgaaaatccattaggaattttcaaccaacgttacaaaaccacactcaggctggctttaaccatgaaatagacttactggttctgagtctagagacagggcaggcttcagatgggtcacggtccagtgggttagtaacacccccaagggcctggtttctttccaggcttcatctctgccttccactgagtcgacaccatcctgagcctctttcctcctatgtggcacagtcttccagcagccctgggccaggggtgggatatgatgacaggtcttttggagaacgtggtggacagttagcaatgtcactcccccacacagtatgtggcaaggaagaagaatctgtgtacacacaaaatctgtctatgaactgagaaaaaacacagggatacccatgacagaccaaggcctgatttccctcgtattgaaagagcttctacaaatcaaccagaaatccaaccaccccacaggtaagtggacaaagaatatggacagttcttgcaaaggaaatactctgtgttccagaaaatccctgtttataaaataaatactataattaaatgtctacatgcattgctgatcagcatcaatttgcccccattgtaactgttatcactatttaaaatagctaacctcggaagagtgccctgagctcacacagcagcacttggtctcctggtcttttctgtcttccctcttgcttatgactttccatgattctcaccatctcatctcataggcaggaactgcacacacgctgcacaggctgcctgttggccactatcagccattcccacccttcccctcctcgcctcagtgacagaggtggctacttccttcccactaggcattatccctgcagggaccccactggggctctgcagattcccagatccctttctctgagtctgccccttccacttggcatgcttttgcttctgacctaaggctcctgcagctcttctgggagggctgttcttgtgctactgcccttttgtgcccacctatagaaagactgaagtacctgggttatcaacgagggtggctcttagccagtggctgacaggcatagaagaatggaagcccagataccctgcctggggcagggacatctcagaggcattgtttacagttgagagctccccttcaggtcaggctgaacctacctgtcatataactgtctgagatccttgcatggctatccttcttctagctccttactgaattctgctcggagcatttcttttaggaacaatctttgtttctgggcctgcttctaggaaacccaacgtaagacacaatcttcttcctcagtaacaaaatcctgagttttattttggcatatggccaccgtgaataaaaactacatttcccagcttcctttgcaaccaagttcttgccaataagatacagggcacaagtgccctgtgagacttctaggaaatccataaagggagtcctgctgatggctagtgtccatcgtggaccctgagggcaaggggtacatcctcaggatgtgggagcagagatctggaaaaggcctggacctctaacaacctcatggatctgccaataccaaccgcagattgtctaccatcccaccattaccccacaacttcttttgagaaataagttcctctcctgtttaagccaatgtcattcgggtgtttattccatgcagttaaatttaatcctagtttacagaccagaccattgactctgaaaaacgacagacactcagtttgccagcctcccttgcagctaggctttgccagtgtaacccagatctggctgaggaggtataaaggaaggtcttggggggaagaaaggtgtaggcaggaggttctggaaaagatatttcttcctgatgcaaaaaacaaacaggtgcacaatgtccagctctctttccactctggcaacctattccctgctacctgcctttggctgcagcatgtgaagatgtgctgtctggagctgtggcagccattctataaccaggaaactacaagtgcatggacaaaaagccaaccagctgaggatggctgtgcagaaggatggagagagcctgggtctttcagaaactcactgagatctcccactccaaaccaataaatggtccacactgttaatcgggttttccattacatacagttgaaagcaatctaacatactcacagggaacaaagcactgaagtaaaatcacctggaagtgatcaattctcaaaaagcctgctactataacctcttggagggtgctatagtttgggtgtttttgtcccctccaaaattcatgttgaaactcaattcccagtgcaagaatgttgggaggtggggcctagagtgaggtgtttaggtcataagagtgggtactctctcactcttccagcatgtgaggacacagcgttcctccccttcataggatgaagcacgcaaagccccattttggaagcagagacagagctaagaccccaccagacaccaagcctgttggtgcctggatcttggacttccaacctccagaactgtgagaaacagatatctgttctttataaattacccagtctcaggtattctattattgcagcacaaaacaaactatggggagatgactgggttctgggaggtgattacctgtgctaggcttgcctctgagggcaagaaacagcaactccagcttcagggaagtgaaataataagaaataaactccaggatccgctgattcctgtgttcaacaatgccatcaggaacccagggccctcccctctctctgctctgccactcttgaaatgggcttcattctcaggcagccagcaagacagaggcatgcttctgggcagcacagccagacctaactggggcctatcgagggcctgcactctcccccttggcttctccctccagctggattttcttgcttttcttcaaacatgccagataggctcctgccctagcctctgcacttgcgttccctctgcctacagtgcttttgcatacatgtccacttggctctgcctccttcaggtcctcacccaaatattacctcccgagagaggcctgccctgaccacaccttttaagattaaccacctcccaactccccatttctttttctggcttaatttttctccctggcatgtaacttcatccaatatagcacacattcccttggcctcactgagtgtccgggccccacttgcctagaaggtgtgctccaggaaggcagagatgtttaagattgttcaccctcattcccccagggcctggcacaggtgtttcacaattatcttcgccctgggggcggaggggaggggcccaccacggccttatttccgcgagcgccggcactgcccgctccgagcccgtgtctgtcgg

SEQ ID NO: 9230 - RNA, 14286 nt, Homo sapiens
  source 1..14286: mol_type = other RNA
agaccctgcagccttcccacccttccccaggccgctctccccagccctggcctcctgcgttcctcttgtgcagcttctctcgggcacagacacaaacctcaccggagttgtgtgggaagatcccaaagcccttcccaatgccaccctgcagggtactgggatgcatgggggtagttgtggcctgtggtcccactcatgcccctgcttcttgtccctcatgtcacttctttcccaggtgaacatggtccttttttgccttcagtccccaaatccacctgtacaaatttgccagatatggcaggctctccatgaaggttttgggataacacagagggagcacagcgtacccaccaaacagaacaaccttgaggtagaatagggtctgaaggcagggaacctaaggctgtttcacattgacttcatagaactaaattgaaaggaaaaccctaactttccatgcctaagtaacaaaaggaccagaggctactccctttgcaaacccccaccttttctacagggcagatgggaaactgaaagtatctctgattggtgccaagcaaccaatcagatgtttgcataggagtgtaacttcataacttcacttcagcctctgactggttgctgtccacagccaatcagactgattgcggaccaagtcttcctttgcataaaagtgcaactttgtaacttcaccttagcctctcatgctaaagtgaatcttaggagtttgcataggagtgtgacccttgtaaccacttcagcctctgagtggaaagcaaccagattgattgcaggccaccacttcatttacatgggtgaacaccaggtggccagtgggaaacctctaggaggtatttggacccaagaagattgtgtatcaggacccttgtgtccctatgctcgggcccacccccacactgtggacagtactttcattttcaataaatctctgcttttgttgcctcactcttcccttactttgtttgtgtgttttgcccaattctttgttcaagatgccaagaacctggacatgcttcaccaacagcaacctgaaattgaaaaccgctaatcattgttcttaaaaggtccttggccatccaagccctgggggttttctactggcagccctgatctcatactcatcccaccaccagtccctgggtcctccccatccttctgctcttatctccactgcttctcctttcccaggctcttcttccctctccagagctaccctgacatttcagtttcatcttcttttattgtactgtgtgtttcagcaatctgagtgttactgtctcccactcatcctcaccttttgaagaaagaaccaaaaacaaaaacaaaaaaagtcaatataggcctttcaagatactccaaaaacttaagaaaaaagtgttaaggctatattacaagaccccagaaaaatgatgctcagaagacaaaagcagtaatttttagtttaaatagtactttttctctggcagtaagtacatcagggagagtcaagacttcctcttggaaaagtatgccatctggttcttgtcatactgttgtgctccttaactcatttcatgcaaaatttccagcaccatgtttgagggaccctgattactcctcatccatgcagtttcagagccacaggagagatgcatgtgggtgggcagaagtggaagttgtttatgagcatgaagtatttctgagaaatgaacgcattgatgttgggatttgaaatctgatttatctctttgatgattacgggaggaaattttattataaacaataatatttgctggcatatgcatggatgtctgaactcagatgataaaaactagaggattttgagcatcttggaaaaaaattgtacaattaatttaagatttcttacatgacctagaaaatgaaaaggggaagcaaatacactggaaaaaaaagaaggtggaggaggatcacattactccttcacagttaattagaagaactttcaaccaaaacacataactgggtaacaaataccaggtaattttctttgactgaattttttttcacttcattttctttgaagtgaaaaaaagtaatttttaaatacaggaaataatattttatgactgagtattctcttcaaagaatctgggtcagcagctcatttcaaattttcagtgcctagaggacgataatacttagtgctgtttgctggtgatttacaacactttcgtggcttaagaccaagaatatacatattaaaaatcatgctctgcctgaatccaacaagcagatgccccaccttcttttaaggaagaacatgacaataatgaacggataatagagtacaaacaaagacactcaaactgcatttcctaatgttgcaaatgttaatattgagtaacaaagcatcatttctattaaagctggccttcagccactcccttatgaggtaggtggaaagaaatctttttactttcccataattctactacttacgggaaagcaagttgactttgcccagcattgatgcaaagagcatgacacagagttcaagccgcagcactgctgctcaggagagtggaaaagagaaaagttattggcacaatagcaaccaagtgtttcatctaaatgttctgtttcttgagctcccaggtaactcagcttcacatcttttccttgtacaggtcaactccacttaggtagaatgtgaatatatagtatgagaggccaaaaacccatacctatataagcaaaattatctccccctactgccaattcataaaaataacacctgccagaatggaacagaatgctgaaaagtctaccttgaaaagatgagcgattttcaagccaagaaaacttgaatgtatgaaaccccctagaaagaatgtgtcatccagggggtaattggcccatcgcagaaacatggaaaagaggaaaaggaagacagcagggcacagtgttcataagaaagagacacaggatgctttttaagaaacttgggtgtgaaagcaaaacaggcaatatttagaaaggaacttttggtcaatgggtggaaatgggttaaaataggagccatttgcacataattatattctaaggggaaggaagcaatagagagagcaattgaaaatgtaaggaagagagggaagaactgatgtgggtgagggtgcatgtttagaacacaggctgggaagagtcggccgcgggagtcacactgctaataaaaggcagagaccaggggtttttggacctgggtgcaaattgtggtcttgccactttctatctgagggaccttgtcaccctgatggtgaaaaacaagcctgtaacagaagaaaggaaagacaagaactgggaggctgtgataagggagctgcatatatcagcagtgcagcaagtctggctgttgacatggttcttggtgagcccaagagagctgactgctggaaaagagtagaggagaacattttcagcctcagaaatatcactggcctctgatgggagagataagtggtctcagggcctaatgagtgctggagaattcattcattcattcagtgaacatgactgaggcctctcactttgctagacattttggaagacaggggtcaaaatcacagttcctactctcaattagctcacagccctgtactagtgatggacaaagaaccagtatgtgacagttcagactaataagcccaacaagagagggatatacaggacactgtgggacccctaaagggagcaccttgtgcagaggtagaaggataggaatgaacgaggggtgacgggtaacaggaagagagagaagcaccgcaggagtctctgaagagtgttcacagggggtgcgaggcttgctgtgcagaaaccaataggggcaggtgagaaatgctgaccccaagggatgagcaggctcatgtcagggtgctacaaccgtcccctcctcttcactctttcctgcaccccagactccaagtcttaaactaggttatctccccagtggcctggcctgccccccgaatgctctcaaaccagtatcttctaaccctagtcaaaaattaccccttcccttcagctagccattagaattgaaacaaattcccactgccatgtgaaagtctgattatcctactgttcccaaggcaccagccttttagtgggatgtttgctgtagtagattgtatcttccaaaaatggccacaaaatgtttctgagtccacatgctcatccagaaactttctactccctcattaagagatagaatctatttcccttccccttgaaattgggctgcctttgtgacttcttcaataaaaagagctgcttggaacccccacccacagcccttacctcccctgcatccatgagcacacccctctgggactatactgtctaccattgcctccctgacttgggactttggctctggagttcactccctaccccaaggccataaaaaacccccactgcactctttagtccctgggctccagccactgccctctccccagatttctctgttttctgccatctctgtgggatccgcataatctgcctccagcagtttctgggagtgaacccagctatcttgctgaaggtagggtaggggtggatgcaacaatgggctgattgttatcaatatgtatggcaagatattatcttgagatattaatctgtgggtttttctttgctcacttccttgtacagtgaccaaacagcctcacgcaagagtacagttggtaaagagggactgaaaagagccaaaaatgtcaacgttcatatttgtgactctaaaacagcatccaagaatcaaaaaagcaaggcttggggcacaaagcacagagacatgtggaccagggacagggatatacagacagccctatcccagtgcctccagggagaccagagtaaggtgtgctgggccgagggaggggaggagcacatggtgaggagcaggtccacattggaagtcttgggagccccaggagcccctcagctggttgcatattcccagagatgtttgccaagccctgattacatatccacactcccctgaatgaacacaccctccccattccagtgtctaaggactctcatgagccctgcagatctgttaggaacactttcagctctaagcaacaaaagatatgattaacagtgccttaaacactacaggtgtattctttcacacaacaagaaggctgtaagtgggtagtttgttggtaaaaatgcagtttatccaggacctagctcatgagcttaggattcaactagttctggaatcatccttaggaatctataattctgaaaacttcctaggtgattctaatttgcaatcagatatggaagccacttctcccaagtttactaaggctgctgtactctcccctcttctgagttttcggagtccattagctttcagaggagtcaacagtgctaccagtgaacacctgactaatttattcactcaaatggtcagcacaccgtaattgctcgctttttacctggtagcatcagctcagtgagggttgtgaactgggcctagagacatgagaattcagcagcatttccaaactgggtagaatttccacagactatttcaagtgctttttttttttccattcaagaaagatggggcaaccagccaagtaaacatggttgtttttgtctgttttgtgttgctaaaacagaatacctgagactgggtaatttataaacgatgatttatttggctcatgttctggaggctggtgctggaatctggtgagggccttctggctatgccattttctggtggaagcgaaagagagagaaaacagggccaaactcatccttttatcaggaacccactcccacagtaactaacccactcccaagataatggcattaagactgtcctgatgacctcatcacctcttaaaggtcccacctgtcaacactgctgcattgaggattaagtttccaacacatgaaacttgagggacacatttaaaccataacaatggtgggctgaacattgtcttttgcctatattcccacccccaaaattcactacagtatcgagattttgttaaaggcaaaaaacaaataaacaaaccatctcaaggacaaggctaaaagagaaaggagcaagtgtggagagagagaggtaaacacgatgtcggaaaccggaaagcaggtggtaaatgatgagtaacttagagaccaggcacaggttgcagagaggaggcaggaagacaacagactggccccggagcacctggtaggcatagaattggaggccccaggaacctctctggttgtggggtgttggttaaaaggctatactaaatacagcttgatcctttgatcgcttctccactcccatcagacaaggcacctctctcatcctacagaagacataccagagaaggggataagggccaagtcagcatgctgaatggcgagaacagcctgcagcctttcgccactgcatctgagaatcctggtgactcagcttagacacatggggcgacaggctacaaatttcttctctggagaaactgagctcctcaaagaaaagacttataaacaatgactactggggattataatcaaatatacatattcagagaaagccaacacagcacaaaaagcagaataaactttaaggaaaactgtaattaatatcttcggagaaagaatataactgcatctacaaaaaagaacaaactactcataaaacaaaaatgagctctcagttctaaaaaaatataaaaacaggaaaaaaaaatccaatagaatccaaacaggctttactgggaaggtactggaggatatattccacaaaatgaaagagcaaaccaggaaaaaggcatacaaaggattcaagagagagggatccaactaaggagaactgaacgacacatcagagcaggaagccaatgggctccagaggggatgtgttaaaaataaaaaatcagttgattacctgatgtgtttgaactattaagaggagattaacactgctggcaatgcgttggaggagaattagggacagaaaaatatcaaaacaagataattttgaactccagggagaaaaagaagttgtataacaacggaagtattatcagtgtacactgtgtgccttaccggggaaaacatttataataatcacaacagttaactttgagtagttacttaattaaaaaatacaatataattacattggaagaataggggaacaaaagtgctcaatcttcatctttcataggaagaagtcaaagtttctgcctaatctgaaaaatcaacacagaagcatataatttagatacctggggaaacatgtggaactttcaactagccgcgccagttgaaaatgggactggtttctctgatgagaatggctgggtaggaaatggtaatctgtcagaccacaaggaatttttctagtcaacaaactccagatgtttgtgattcttttcctcctggttcactgggttcagccaaagtcctccctagaagattgccaagtgtaagctgagcttgaatctgttccgtgctcccttcttactgatacaacctcgaccagttacttaattctctgtggcacccagtttagtcctcaaacttgtggagattaaacaagattattctcggatcacacaggtcaagcagggctataaaaccgggcagcctggctccaagtctactctctgagccactgtgcaacctacaaacgataacagaaaagaacccaaagacttaacagttagagaaagcccctctgaccccaagcattctctctgttcccctaaccattgttagtcatttctgatttgtccttccagagacagtctgtgtgcacatctttctaaatgcacatctagaaagaagaagcttctgatatcaccttgggcagtcacactcatgcacaaataggagatgtttttatcttttctaataactgatatcaactttgctttccaagtccctatttgggtgcttacactggtgagtgcaggggcaaggacagaggagaaaatagtctcaacgaagggtacctttgcaaaatactccatccaccccagtgtttctgctgtcttctctgatgtgactctcagccatgatgtaggttaaagcgtctatcttagggattccttctccttccccagggtcttttttcctctctccccacaaccctgctctccctcacagccttagagagggcagcagggcttgtggagctcagagacgatgctcaaatgggaacagacaattgtccagcgtggaagcagtcacttctgacctggggtcatggcttggcctggcccctgtggctgacaaggcactactgccatggctgggagttgctggtgaaaggaaatgtcccttctccagctgggtcatcccaaaattggtggactctgaagatatggtagtcccagtgcaggtagcagctgtggtgttcccagattgtttggcttccaccacacccggcactatctccccactgcctcccacctcccacccccagtacgaggcagccttagatctctgtgtttcctgccaatactaactgcctgttggatgaaaatccattaggaattttcaaccaacgttacaaaaccacactcaggctggctttaaccatgaaatagacttactggttctgagtctagagacagggcaggcttcagatgggtcacggtccagtgggttagtaacacccccaagggcctggtttctttccaggcttcatctctgccttccactgagtcgacaccatcctgagcctctttcctgagggaggcaagatggcaccaccagcttctggggcacacacttcctctcacatgcacggtagaggaagggagagcacacactctcagaagagcaagacaacttccctccaagactccaccaaccgcttctcctgacttacttgcccaaatagggtcctgagcctatccctgaacccaccacagtgacactgtctctctccagtcagattgccagaatgaggtgtgttcagcagcactggagagaggtgagcaaaggtgaaaatcagagcagcattagcaggaagaggggacagctgctgggaggccccccgcacacctgcgtccacatgccctcacctgttcttgatgtattctcagggcttggctaagagaacctggggcctgagatgcttgggaactggctcctgggccttcttacattccacaagctggggtggccaaaggtaaccaggatggcagtgtcactatgaccttctttctccgcagccaaccacctggtctcctcatgcccagtcctctcatctgctgcgaagacacatcccaggccctctgggacgggtttgctatagactgaattgtgtccccccagttcatgtgttgaagccctaacctccaatgtgatggtatttggaggtggggcctttgggaggcgattacagttagatgaagtctaaccataattactaatcccatgatgggattagtgtccttataagaagagacacagaggcttgccgcttccctctctgctgtgtgagcatgcagtttcaggccacgtcaggaagaggggcctcggcaggaactgaatcagccagcatcttgatcttggacttcccagcttccaatccatcgaaaacacatttctgttgtttaagccacccagtttgtggtattttgttatggcagaacaagttggttaagacaaggaaaataaacagccaatgcctctcagagccctctctctctgctctctggcctctttatgtagtcaagaggataggaggggggcaagtacagctgttcaggggctgctggatacgtctacctagcatagggcacagaagccaatgctgcaatctgctcagtcagaacttaggtctcttggctcaagacctggtccctatttaaataacagtacttccaagatgagcaatgcagtgagccgtggcagccactgacactacagtacgaatctgctcagcagctccttccctggaagtttcagtgtgaggaaacatgactaggtccgaggcaagaaagagtgtggcgaggcaagactcagagaaagggagacaagctggaactacacaacaagcaagcaaggcaggcaggctctggctacgcagaacgacagcactgtaaagctcctgtggcggtcttccctaccggaggagaaactgattgaagcgcattcggaaacagcacctcatttatttacttatttagaatagacaatatacattatacacacatgaaaaaagcaaccaccacaaaagagagccaatggtgaagagtttctctctcatcctatattggcaattcttataaacctttgcagagacagtttttgcatatttccacatttatgtatgttatttttttctttttaaacaaatagcagcatactacttgccctactctacaccttgctgttaacaacattataccttagagatggttcagtatcacacacacctcaatctacctcttcttcatgactgtacaatattccattctatggaggtactataattagtcaaccatgaaacacaggtgttttcccagcccttaactcttcattgtttaaaaaaaaaaatctgtattcgtgtctattgtgtgccagtcactgttctagggaatagagagtagaaaatgagacattcagtgtcactgccgtggaggagtttacaatccatatgtggaaatgaacatccttgcacatacttctttatgtacatgtgtgaatgtattgttattataaactctcaaggtggaattgctgggtcagagccatgtgcatttctaatttcaatagatattgcaaattgtccaccaaacaggtcatgtcagtttcccctctcaccgtctgtactatcttttcatatgattaaaagtcattatagctttatataccattaggtttcttaaacacaaagtaagttctctaaaatgctcatgataacctgagcaatgactaaggaactagggaacatgacatatcaggacacccttgtggggacacatctgcttctgtgcagaggctggggcagaacctgctggctgatactttcctcacctcctatgtggcacagtcttccagcagccctgggccaggggtgggatatgatgacaggtcttttggagaacgtggtggacagttagcaatgtcactcccccacacagtatgtggcaaggaagaagaatctgtgtacacacaaaatctgtctatgaactgagaaaaaacacagggatacccatgacagaccaaggcctgatttccctcgtattgaaagagcttctacaaatcaaccagaaatccaaccaccccacaggtaagtggacaaagaatatggacagttcttgcaaaggaaatactctgtgttccagaaaatccctgtttataaaataaatactataattaaatgtctacatgcattgctgatcagcatcaatttgcccccattgtaactgttatcactatttaaaatagctaacctcggaagagtgccctgagctcacacagcagcacttggtctcctggtcttttctgtcttccctcttgcttatgactttccatgattctcaccatctcatctcataggcaggaactgcacacacgctgcacaggctgcctgttggccactatcagccattcccacccttcccctcctcgcctcagtgacagaggtggctacttccttcccactaggcattatccctgcagggaccccactggggctctgcagattcccagatccctttctctgagtctgccccttccacttggcatgcttttgcttctgacctaaggctcctgcagctcttctgggagggctgttcttgtgctactgcccttttgtgcccacctatagaaagactgaagtacctgggttatcaacgagggtggctcttagccagtggctgacaggcatagaagaatggaagcccagataccctgcctggggcagggacatctcagaggcattgtttacagttgagagctccccttcaggtcaggctgaacctacctgtcatataactgtctgagatccttgcatggctatccttcttctagctccttactgaattctgctcggagcatttcttttaggaacaatctttgtttctgggcctgcttctaggaaacccaacgtaagacacaatcttcttcctcagtaacaaaatcctgagttttattttggcatatggccaccgtgaataaaaactacatttcccagcttcctttgcaaccaagttcttgccaataagatacagggcacaagtgccctgtgagacttctaggaaatccataaagggagtcctgctgatggctagtgtccatcgtggaccctgagggcaaggggtacatcctcaggatgtgggagcagagatctggaaaaggcctggacctctaacaacctcatggatctgccaataccaaccgcagattgtctaccatcccaccattaccccacaacttcttttgagaaataagttcctctcctgtttaagccaatgtcattcgggtgtttattccatgcagttaaatttaatcctagtttacagaccagaccattgactctgaaaaacgacagacactcagtttgccagcctcccttgcagctaggctttgccagtgtaacccagatctggctgaggaggtataaaggaaggtcttggggggaagaaaggtgtaggcaggaggttctggaaaagatatttcttcctgatgcaaaaaacaaacaggtgcacaatgtccagctctctttccactctggcaacctattccctgctacctgcctttggctgcagcatgtgaagatgtgctgtctggagctgtggcagccattctataaccaggaaactacaagtgcatggacaaaaagccaaccagctgaggatggctgtgcagaaggatggagagagcctgggtctttcagaaactcactgagatctcccactccaaaccaataaatggtccacactgttaatcgggttttccattacatacagttgaaagcaatctaacatactcacagggaacaaagcactgaagtaaaatcacctggaagtgatcaattctcaaaaagcctgctactataacctcttggagggtgctatagtttgggtgtttttgtcccctccaaaattcatgttgaaactcaattcccagtgcaagaatgttgggaggtggggcctagagtgaggtgtttaggtcataagagtgggtactctctcactcttccagcatgtgaggacacagcgttcctccccttcataggatgaagcacgcaaagccccattttggaagcagagacagagctaagaccccaccagacaccaagcctgttggtgcctggatcttggacttccaacctccagaactgtgagaaacagatatctgttctttataaattacccagtctcaggtattctattattgcagcacaaaacaaactatggggagatgactgggttctgggaggtgattacctgtgctaggcttgcctctgagggcaagaaacagcaactccagcttcagggaagtgaaataataagaaataaactccaggatccgctgattcctgtgttcaacaatgccatcaggaacccagggccctcccctctctctgctctgccactcttgaaatgggcttcattctcaggcagccagcaagacagaggcatgcttctgggcagcacagccagacctaactggggcctatcgagggcctgcactctcccccttggcttctccctccagctggattttcttgcttttcttcaaacatgccagataggctcctgccctagcctctgcacttgcgttccctctgcctacagtgcttttgcatacatgtccacttggctctgcctccttcaggtcctcacccaaatattacctcccgagagaggcctgccctgaccacaccttttaagattaaccacctcccaactccccatttctttttctggcttaatttttctccctggcatgtaacttcatccaatatagcacacattcccttggcctcactgagtgtccgggccccacttgcctagaaggtgtgctccaggaaggcagagatgtttaagattgttcaccctcattcccccagggcctggcacaggtgtttcacaattatcctgccttgctgcccactcctccctcctcggcgcctcttctgggcaggaccggcaggtgttcaggcccgtccccagcccctggctccggcgtcccgggctccctgccggcatccaccttcacctcctccccagccccagccctctggcgact

SEQ ID NO: 9231 - RNA, 14284 nt, Homo sapiens
  source 1..14284: mol_type = other RNA
agaccctgcagccttcccacccttccccaggccgctctccccagccctggcctcctgcgttcctcttgtgcagcttctctcgggcacagacacaaacctcaccggagttgtgtgggaagatcccaaagcccttcccaatgccaccctgcagggtactgggatgcatgggggtagttgtggcctgtggtcccactcatgcccctgcttcttgtccctcatgtcacttctttcccaggtgaacatggtccttttttgccttcagtccccaaatccacctgtacaaatttgccagatatggcaggctctccatgaaggttttgggataacacagagggagcacagcgtacccaccaaacagaacaaccttgaggtagaatagggtctgaaggcagggaacctaaggctgtttcacattgacttcatagaactaaattgaaaggaaaaccctaactttccatgcctaagtaacaaaaggaccagaggctactccctttgcaaacccccaccttttctacagggcagatgggaaactgaaagtatctctgattggtgccaagcaaccaatcagatgtttgcataggagtgtaacttcataacttcacttcagcctctgactggttgctgtccacagccaatcagactgattgcggaccaagtcttcctttgcataaaagtgcaactttgtaacttcaccttagcctctcatgctaaagtgaatcttaggagtttgcataggagtgtgacccttgtaaccacttcagcctctgagtggaaagcaaccagattgattgcaggccaccacttcatttacatgggtgaacaccaggtggccagtgggaaacctctaggaggtatttggacccaagaagattgtgtatcaggacccttgtgtccctatgctcgggcccacccccacactgtggacagtactttcattttcaataaatctctgcttttgttgcctcactcttcccttactttgtttgtgtgttttgcccaattctttgttcaagatgccaagaacctggacatgcttcaccaacagcaacctgaaattgaaaaccgctaatcattgttcttaaaaggtccttggccatccaagccctgggggttttctactggcagccctgatctcatactcatcccaccaccagtccctgggtcctccccatccttctgctcttatctccactgcttctcctttcccaggctcttcttccctctccagagctaccctgacatttcagtttcatcttcttttattgtactgtgtgtttcagcaatctgagtgttactgtctcccactcatcctcaccttttgaagaaagaaccaaaaacaaaaacaaaaaaagtcaatataggcctttcaagatactccaaaaacttaagaaaaaagtgttaaggctatattacaagaccccagaaaaatgatgctcagaagacaaaagcagtaatttttagtttaaatagtactttttctctggcagtaagtacatcagggagagtcaagacttcctcttggaaaagtatgccatctggttcttgtcatactgttgtgctccttaactcatttcatgcaaaatttccagcaccatgtttgagggaccctgattactcctcatccatgcagtttcagagccacaggagagatgcatgtgggtgggcagaagtggaagttgtttatgagcatgaagtatttctgagaaatgaacgcattgatgttgggatttgaaatctgatttatctctttgatgattacgggaggaaattttattataaacaataatatttgctggcatatgcatggatgtctgaactcagatgataaaaactagaggattttgagcatcttggaaaaaaattgtacaattaatttaagatttcttacatgacctagaaaatgaaaaggggaagcaaatacactggaaaaaaaagaaggtggaggaggatcacattactccttcacagttaattagaagaactttcaaccaaaacacataactgggtaacaaataccaggtaattttctttgactgaattttttttcacttcattttctttgaagtgaaaaaaagtaatttttaaatacaggaaataatattttatgactgagtattctcttcaaagaatctgggtcagcagctcatttcaaattttcagtgcctagaggacgataatacttagtgctgtttgctggtgatttacaacactttcgtggcttaagaccaagaatatacatattaaaaatcatgctctgcctgaatccaacaagcagatgccccaccttcttttaaggaagaacatgacaataatgaacggataatagagtacaaacaaagacactcaaactgcatttcctaatgttgcaaatgttaatattgagtaacaaagcatcatttctattaaagctggccttcagccactcccttatgaggtaggtggaaagaaatctttttactttcccataattctactacttacgggaaagcaagttgactttgcccagcattgatgcaaagagcatgacacagagttcaagccgcagcactgctgctcaggagagtggaaaagagaaaagttattggcacaatagcaaccaagtgtttcatctaaatgttctgtttcttgagctcccaggtaactcagcttcacatcttttccttgtacaggtcaactccacttaggtagaatgtgaatatatagtatgagaggccaaaaacccatacctatataagcaaaattatctccccctactgccaattcataaaaataacacctgccagaatggaacagaatgctgaaaagtctaccttgaaaagatgagcgattttcaagccaagaaaacttgaatgtatgaaaccccctagaaagaatgtgtcatccagggggtaattggcccatcgcagaaacatggaaaagaggaaaaggaagacagcagggcacagtgttcataagaaagagacacaggatgctttttaagaaacttgggtgtgaaagcaaaacaggcaatatttagaaaggaacttttggtcaatgggtggaaatgggttaaaataggagccatttgcacataattatattctaaggggaaggaagcaatagagagagcaattgaaaatgtaaggaagagagggaagaactgatgtgggtgagggtgcatgtttagaacacaggctgggaagagtcggccgcgggagtcacactgctaataaaaggcagagaccaggggtttttggacctgggtgcaaattgtggtcttgccactttctatctgagggaccttgtcaccctgatggtgaaaaacaagcctgtaacagaagaaaggaaagacaagaactgggaggctgtgataagggagctgcatatatcagcagtgcagcaagtctggctgttgacatggttcttggtgagcccaagagagctgactgctggaaaagagtagaggagaacattttcagcctcagaaatatcactggcctctgatgggagagataagtggtctcagggcctaatgagtgctggagaattcattcattcattcagtgaacatgactgaggcctctcactttgctagacattttggaagacaggggtcaaaatcacagttcctactctcaattagctcacagccctgtactagtgatggacaaagaaccagtatgtgacagttcagactaataagcccaacaagagagggatatacaggacactgtgggacccctaaagggagcaccttgtgcagaggtagaaggataggaatgaacgaggggtgacgggtaacaggaagagagagaagcaccgcaggagtctctgaagagtgttcacagggggtgcgaggcttgctgtgcagaaaccaataggggcaggtgagaaatgctgaccccaagggatgagcaggctcatgtcagggtgctacaaccgtcccctcctcttcactctttcctgcaccccagactccaagtcttaaactaggttatctccccagtggcctggcctgccccccgaatgctctcaaaccagtatcttctaaccctagtcaaaaattaccccttcccttcagctagccattagaattgaaacaaattcccactgccatgtgaaagtctgattatcctactgttcccaaggcaccagccttttagtgggatgtttgctgtagtagattgtatcttccaaaaatggccacaaaatgtttctgagtccacatgctcatccagaaactttctactccctcattaagagatagaatctatttcccttccccttgaaattgggctgcctttgtgacttcttcaataaaaagagctgcttggaacccccacccacagcccttacctcccctgcatccatgagcacacccctctgggactatactgtctaccattgcctccctgacttgggactttggctctggagttcactccctaccccaaggccataaaaaacccccactgcactctttagtccctgggctccagccactgccctctccccagatttctctgttttctgccatctctgtgggatccgcataatctgcctccagcagtttctgggagtgaacccagctatcttgctgaaggtagggtaggggtggatgcaacaatgggctgattgttatcaatatgtatggcaagatattatcttgagatattaatctgtgggtttttctttgctcacttccttgtacagtgaccaaacagcctcacgcaagagtacagttggtaaagagggactgaaaagagccaaaaatgtcaacgttcatatttgtgactctaaaacagcatccaagaatcaaaaaagcaaggcttggggcacaaagcacagagacatgtggaccagggacagggatatacagacagccctatcccagtgcctccagggagaccagagtaaggtgtgctgggccgagggaggggaggagcacatggtgaggagcaggtccacattggaagtcttgggagccccaggagcccctcagctggttgcatattcccagagatgtttgccaagccctgattacatatccacactcccctgaatgaacacaccctccccattccagtgtctaaggactctcatgagccctgcagatctgttaggaacactttcagctctaagcaacaaaagatatgattaacagtgccttaaacactacaggtgtattctttcacacaacaagaaggctgtaagtgggtagtttgttggtaaaaatgcagtttatccaggacctagctcatgagcttaggattcaactagttctggaatcatccttaggaatctataattctgaaaacttcctaggtgattctaatttgcaatcagatatggaagccacttctcccaagtttactaaggctgctgtactctcccctcttctgagttttcggagtccattagctttcagaggagtcaacagtgctaccagtgaacacctgactaatttattcactcaaatggtcagcacaccgtaattgctcgctttttacctggtagcatcagctcagtgagggttgtgaactgggcctagagacatgagaattcagcagcatttccaaactgggtagaatttccacagactatttcaagtgctttttttttttccattcaagaaagatggggcaaccagccaagtaaacatggttgtttttgtctgttttgtgttgctaaaacagaatacctgagactgggtaatttataaacgatgatttatttggctcatgttctggaggctggtgctggaatctggtgagggccttctggctatgccattttctggtggaagcgaaagagagagaaaacagggccaaactcatccttttatcaggaacccactcccacagtaactaacccactcccaagataatggcattaagactgtcctgatgacctcatcacctcttaaaggtcccacctgtcaacactgctgcattgaggattaagtttccaacacatgaaacttgagggacacatttaaaccataacaatggtgggctgaacattgtcttttgcctatattcccacccccaaaattcactacagtatcgagattttgttaaaggcaaaaaacaaataaacaaaccatctcaaggacaaggctaaaagagaaaggagcaagtgtggagagagagaggtaaacacgatgtcggaaaccggaaagcaggtggtaaatgatgagtaacttagagaccaggcacaggttgcagagaggaggcaggaagacaacagactggccccggagcacctggtaggcatagaattggaggccccaggaacctctctggttgtggggtgttggttaaaaggctatactaaatacagcttgatcctttgatcgcttctccactcccatcagacaaggcacctctctcatcctacagaagacataccagagaaggggataagggccaagtcagcatgctgaatggcgagaacagcctgcagcctttcgccactgcatctgagaatcctggtgactcagcttagacacatggggcgacaggctacaaatttcttctctggagaaactgagctcctcaaagaaaagacttataaacaatgactactggggattataatcaaatatacatattcagagaaagccaacacagcacaaaaagcagaataaactttaaggaaaactgtaattaatatcttcggagaaagaatataactgcatctacaaaaaagaacaaactactcataaaacaaaaatgagctctcagttctaaaaaaatataaaaacaggaaaaaaaaatccaatagaatccaaacaggctttactgggaaggtactggaggatatattccacaaaatgaaagagcaaaccaggaaaaaggcatacaaaggattcaagagagagggatccaactaaggagaactgaacgacacatcagagcaggaagccaatgggctccagaggggatgtgttaaaaataaaaaatcagttgattacctgatgtgtttgaactattaagaggagattaacactgctggcaatgcgttggaggagaattagggacagaaaaatatcaaaacaagataattttgaactccagggagaaaaagaagttgtataacaacggaagtattatcagtgtacactgtgtgccttaccggggaaaacatttataataatcacaacagttaactttgagtagttacttaattaaaaaatacaatataattacattggaagaataggggaacaaaagtgctcaatcttcatctttcataggaagaagtcaaagtttctgcctaatctgaaaaatcaacacagaagcatataatttagatacctggggaaacatgtggaactttcaactagccgcgccagttgaaaatgggactggtttctctgatgagaatggctgggtaggaaatggtaatctgtcagaccacaaggaatttttctagtcaacaaactccagatgtttgtgattcttttcctcctggttcactgggttcagccaaagtcctccctagaagattgccaagtgtaagctgagcttgaatctgttccgtgctcccttcttactgatacaacctcgaccagttacttaattctctgtggcacccagtttagtcctcaaacttgtggagattaaacaagattattctcggatcacacaggtcaagcagggctataaaaccgggcagcctggctccaagtctactctctgagccactgtgcaacctacaaacgataacagaaaagaacccaaagacttaacagttagagaaagcccctctgaccccaagcattctctctgttcccctaaccattgttagtcatttctgatttgtccttccagagacagtctgtgtgcacatctttctaaatgcacatctagaaagaagaagcttctgatatcaccttgggcagtcacactcatgcacaaataggagatgtttttatcttttctaataactgatatcaactttgctttccaagtccctatttgggtgcttacactggtgagtgcaggggcaaggacagaggagaaaatagtctcaacgaagggtacctttgcaaaatactccatccaccccagtgtttctgctgtcttctctgatgtgactctcagccatgatgtaggttaaagcgtctatcttagggattccttctccttccccagggtcttttttcctctctccccacaaccctgctctccctcacagccttagagagggcagcagggcttgtggagctcagagacgatgctcaaatgggaacagacaattgtccagcgtggaagcagtcacttctgacctggggtcatggcttggcctggcccctgtggctgacaaggcactactgccatggctgggagttgctggtgaaaggaaatgtcccttctccagctgggtcatcccaaaattggtggactctgaagatatggtagtcccagtgcaggtagcagctgtggtgttcccagattgtttggcttccaccacacccggcactatctccccactgcctcccacctcccacccccagtacgaggcagccttagatctctgtgtttcctgccaatactaactgcctgttggatgaaaatccattaggaattttcaaccaacgttacaaaaccacactcaggctggctttaaccatgaaatagacttactggttctgagtctagagacagggcaggcttcagatgggtcacggtccagtgggttagtaacacccccaagggcctggtttctttccaggcttcatctctgccttccactgagtcgacaccatcctgagcctctttcctgagggaggcaagatggcaccaccagcttctggggcacacacttcctctcacatgcacggtagaggaagggagagcacacactctcagaagagcaagacaacttccctccaagactccaccaaccgcttctcctgacttacttgcccaaatagggtcctgagcctatccctgaacccaccacagtgacactgtctctctccagtcagattgccagaatgaggtgtgttcagcagcactggagagaggtgagcaaaggtgaaaatcagagcagcattagcaggaagaggggacagctgctgggaggccccccgcacacctgcgtccacatgccctcacctgttcttgatgtattctcagggcttggctaagagaacctggggcctgagatgcttgggaactggctcctgggccttcttacattccacaagctggggtggccaaaggtaaccaggatggcagtgtcactatgaccttctttctccgcagccaaccacctggtctcctcatgcccagtcctctcatctgctgcgaagacacatcccaggccctctgggacgggtttgctatagactgaattgtgtccccccagttcatgtgttgaagccctaacctccaatgtgatggtatttggaggtggggcctttgggaggcgattacagttagatgaagtctaaccataattactaatcccatgatgggattagtgtccttataagaagagacacagaggcttgccgcttccctctctgctgtgtgagcatgcagtttcaggccacgtcaggaagaggggcctcggcaggaactgaatcagccagcatcttgatcttggacttcccagcttccaatccatcgaaaacacatttctgttgtttaagccacccagtttgtggtattttgttatggcagaacaagttggttaagacaaggaaaataaacagccaatgcctctcagagccctctctctctgctctctggcctctttatgtagtcaagaggataggaggggggcaagtacagctgttcaggggctgctggatacgtctacctagcatagggcacagaagccaatgctgcaatctgctcagtcagaacttaggtctcttggctcaagacctggtccctatttaaataacagtacttccaagatgagcaatgcagtgagccgtggcagccactgacactacagtacgaatctgctcagcagctccttccctggaagtttcagtgtgaggaaacatgactaggtccgaggcaagaaagagtgtggcgaggcaagactcagagaaagggagacaagctggaactacacaacaagcaagcaaggcaggcaggctctggctacgcagaacgacagcactgtaaagctcctgtggcggtcttccctaccggaggagaaactgattgaagcgcattcggaaacagcacctcatttatttacttatttagaatagacaatatacattatacacacatgaaaaaagcaaccaccacaaaagagagccaatggtgaagagtttctctctcatcctatattggcaattcttataaacctttgcagagacagtttttgcatatttccacatttatgtatgttatttttttctttttaaacaaatagcagcatactacttgccctactctacaccttgctgttaacaacattataccttagagatggttcagtatcacacacacctcaatctacctcttcttcatgactgtacaatattccattctatggaggtactataattagtcaaccatgaaacacaggtgttttcccagcccttaactcttcattgtttaaaaaaaaaaatctgtattcgtgtctattgtgtgccagtcactgttctagggaatagagagtagaaaatgagacattcagtgtcactgccgtggaggagtttacaatccatatgtggaaatgaacatccttgcacatacttctttatgtacatgtgtgaatgtattgttattataaactctcaaggtggaattgctgggtcagagccatgtgcatttctaatttcaatagatattgcaaattgtccaccaaacaggtcatgtcagtttcccctctcaccgtctgtactatcttttcatatgattaaaagtcattatagctttatataccattaggtttcttaaacacaaagtaagttctctaaaatgctcatgataacctgagcaatgactaaggaactagggaacatgacatatcaggacacccttgtggggacacatctgcttctgtgcagaggctggggcagaacctgctggctgatactttcctcacctcctatgtggcacagtcttccagcagccctgggccaggggtgggatatgatgacaggtcttttggagaacgtggtggacagttagcaatgtcactcccccacacagtatgtggcaaggaagaagaatctgtgtacacacaaaatctgtctatgaactgagaaaaaacacagggatacccatgacagaccaaggcctgatttccctcgtattgaaagagcttctacaaatcaaccagaaatccaaccaccccacaggtaagtggacaaagaatatggacagttcttgcaaaggaaatactctgtgttccagaaaatccctgtttataaaataaatactataattaaatgtctacatgcattgctgatcagcatcaatttgcccccattgtaactgttatcactatttaaaatagctaacctcggaagagtgccctgagctcacacagcagcacttggtctcctggtcttttctgtcttccctcttgcttatgactttccatgattctcaccatctcatctcataggcaggaactgcacacacgctgcacaggctgcctgttggccactatcagccattcccacccttcccctcctcgcctcagtgacagaggtggctacttccttcccactaggcattatccctgcagggaccccactggggctctgcagattcccagatccctttctctgagtctgccccttccacttggcatgcttttgcttctgacctaaggctcctgcagctcttctgggagggctgttcttgtgctactgcccttttgtgcccacctatagaaagactgaagtacctgggttatcaacgagggtggctcttagccagtggctgacaggcatagaagaatggaagcccagataccctgcctggggcagggacatctcagaggcattgtttacagttgagagctccccttcaggtcaggctgaacctacctgtcatataactgtctgagatccttgcatggctatccttcttctagctccttactgaattctgctcggagcatttcttttaggaacaatctttgtttctgggcctgcttctaggaaacccaacgtaagacacaatcttcttcctcagtaacaaaatcctgagttttattttggcatatggccaccgtgaataaaaactacatttcccagcttcctttgcaaccaagttcttgccaataagatacagggcacaagtgccctgtgagacttctaggaaatccataaagggagtcctgctgatggctagtgtccatcgtggaccctgagggcaaggggtacatcctcaggatgtgggagcagagatctggaaaaggcctggacctctaacaacctcatggatctgccaataccaaccgcagattgtctaccatcccaccattaccccacaacttcttttgagaaataagttcctctcctgtttaagccaatgtcattcgggtgtttattccatgcagttaaatttaatcctagtttacagaccagaccattgactctgaaaaacgacagacactcagtttgccagcctcccttgcagctaggctttgccagtgtaacccagatctggctgaggaggtataaaggaaggtcttggggggaagaaaggtgtaggcaggaggttctggaaaagatatttcttcctgatgcaaaaaacaaacaggtgcacaatgtccagctctctttccactctggcaacctattccctgctacctgcctttggctgcagcatgtgaagatgtgctgtctggagctgtggcagccattctataaccaggaaactacaagtgcatggacaaaaagccaaccagctgaggatggctgtgcagaaggatggagagagcctgggtctttcagaaactcactgagatctcccactccaaaccaataaatggtccacactgttaatcgggttttccattacatacagttgaaagcaatctaacatactcacagggaacaaagcactgaagtaaaatcacctggaagtgatcaattctcaaaaagcctgctactataacctcttggagggtgctatagtttgggtgtttttgtcccctccaaaattcatgttgaaactcaattcccagtgcaagaatgttgggaggtggggcctagagtgaggtgtttaggtcataagagtgggtactctctcactcttccagcatgtgaggacacagcgttcctccccttcataggatgaagcacgcaaagccccattttggaagcagagacagagctaagaccccaccagacaccaagcctgttggtgcctggatcttggacttccaacctccagaactgtgagaaacagatatctgttctttataaattacccagtctcaggtattctattattgcagcacaaaacaaactatggggagatgactgggttctgggaggtgattacctgtgctaggcttgcctctgagggcaagaaacagcaactccagcttcagggaagtgaaataataagaaataaactccaggatccgctgattcctgtgttcaacaatgccatcaggaacccagggccctcccctctctctgctctgccactcttgaaatgggcttcattctcaggcagccagcaagacagaggcatgcttctgggcagcacagccagacctaactggggcctatcgagggcctgcactctcccccttggcttctccctccagctggattttcttgcttttcttcaaacatgccagataggctcctgccctagcctctgcacttgcgttccctctgcctacagtgcttttgcatacatgtccacttggctctgcctccttcaggtcctcacccaaatattacctcccgagagaggcctgccctgaccacaccttttaagattaaccacctcccaactccccatttctttttctggcttaatttttctccctggcatgtaacttcatccaatatagcacacattcccttggcctcactgagtgtccgggccccacttgcctagaaggtgtgctccaggaaggcagagatgtttaagattgttcaccctcattcccccagggcctggcacaggtgtttcacaattatctccacagtggctgtgccacgaggagccccatcaatgcccgctgcggcctgcccctttctccgccgtcccctttcacctgcttcgccctgggggcggaggggaggggcccaccacggccttatttccgcgagcgccggcactgcccgctc

SEQ ID NO: 9232 - RNA, 14287 nt, Homo sapiens
  source 1..14287: mol_type = other RNA
agaccctgcagccttcccacccttccccaggccgctctccccagccctggcctcctgcgttcctcttgtgcagcttctctcgggcacagacacaaacctcaccggagttgtgtgggaagatcccaaagcccttcccaatgccaccctgcagggtactgggatgcatgggggtagttgtggcctgtggtcccactcatgcccctgcttcttgtccctcatgtcacttctttcccaggtgaacatggtccttttttgccttcagtccccaaatccacctgtacaaatttgccagatatggcaggctctccatgaaggttttgggataacacagagggagcacagcgtacccaccaaacagaacaaccttgaggtagaatagggtctgaaggcagggaacctaaggctgtttcacattgacttcatagaactaaattgaaaggaaaaccctaactttccatgcctaagtaacaaaaggaccagaggctactccctttgcaaacccccaccttttctacagggcagatgggaaactgaaagtatctctgattggtgccaagcaaccaatcagatgtttgcataggagtgtaacttcataacttcacttcagcctctgactggttgctgtccacagccaatcagactgattgcggaccaagtcttcctttgcataaaagtgcaactttgtaacttcaccttagcctctcatgctaaagtgaatcttaggagtttgcataggagtgtgacccttgtaaccacttcagcctctgagtggaaagcaaccagattgattgcaggccaccacttcatttacatgggtgaacaccaggtggccagtgggaaacctctaggaggtatttggacccaagaagattgtgtatcaggacccttgtgtccctatgctcgggcccacccccacactgtggacagtactttcattttcaataaatctctgcttttgttgcctcactcttcccttactttgtttgtgtgttttgcccaattctttgttcaagatgccaagaacctggacatgcttcaccaacagcaacctgaaattgaaaaccgctaatcattgttcttaaaaggtccttggccatccaagccctgggggttttctactggcagccctgatctcatactcatcccaccaccagtccctgggtcctccccatccttctgctcttatctccactgcttctcctttcccaggctcttcttccctctccagagctaccctgacatttcagtttcatcttcttttattgtactgtgtgtttcagcaatctgagtgttactgtctcccactcatcctcaccttttgaagaaagaaccaaaaacaaaaacaaaaaaagtcaatataggcctttcaagatactccaaaaacttaagaaaaaagtgttaaggctatattacaagaccccagaaaaatgatgctcagaagacaaaagcagtaatttttagtttaaatagtactttttctctggcagtaagtacatcagggagagtcaagacttcctcttggaaaagtatgccatctggttcttgtcatactgttgtgctccttaactcatttcatgcaaaatttccagcaccatgtttgagggaccctgattactcctcatccatgcagtttcagagccacaggagagatgcatgtgggtgggcagaagtggaagttgtttatgagcatgaagtatttctgagaaatgaacgcattgatgttgggatttgaaatctgatttatctctttgatgattacgggaggaaattttattataaacaataatatttgctggcatatgcatggatgtctgaactcagatgataaaaactagaggattttgagcatcttggaaaaaaattgtacaattaatttaagatttcttacatgacctagaaaatgaaaaggggaagcaaatacactggaaaaaaaagaaggtggaggaggatcacattactccttcacagttaattagaagaactttcaaccaaaacacataactgggtaacaaataccaggtaattttctttgactgaattttttttcacttcattttctttgaagtgaaaaaaagtaatttttaaatacaggaaataatattttatgactgagtattctcttcaaagaatctgggtcagcagctcatttcaaattttcagtgcctagaggacgataatacttagtgctgtttgctggtgatttacaacactttcgtggcttaagaccaagaatatacatattaaaaatcatgctctgcctgaatccaacaagcagatgccccaccttcttttaaggaagaacatgacaataatgaacggataatagagtacaaacaaagacactcaaactgcatttcctaatgttgcaaatgttaatattgagtaacaaagcatcatttctattaaagctggccttcagccactcccttatgaggtaggtggaaagaaatctttttactttcccataattctactacttacgggaaagcaagttgactttgcccagcattgatgcaaagagcatgacacagagttcaagccgcagcactgctgctcaggagagtggaaaagagaaaagttattggcacaatagcaaccaagtgtttcatctaaatgttctgtttcttgagctcccaggtaactcagcttcacatcttttccttgtacaggtcaactccacttaggtagaatgtgaatatatagtatgagaggccaaaaacccatacctatataagcaaaattatctccccctactgccaattcataaaaataacacctgccagaatggaacagaatgctgaaaagtctaccttgaaaagatgagcgattttcaagccaagaaaacttgaatgtatgaaaccccctagaaagaatgtgtcatccagggggtaattggcccatcgcagaaacatggaaaagaggaaaaggaagacagcagggcacagtgttcataagaaagagacacaggatgctttttaagaaacttgggtgtgaaagcaaaacaggcaatatttagaaaggaacttttggtcaatgggtggaaatgggttaaaataggagccatttgcacataattatattctaaggggaaggaagcaatagagagagcaattgaaaatgtaaggaagagagggaagaactgatgtgggtgagggtgcatgtttagaacacaggctgggaagagtcggccgcgggagtcacactgctaataaaaggcagagaccaggggtttttggacctgggtgcaaattgtggtcttgccactttctatctgagggaccttgtcaccctgatggtgaaaaacaagcctgtaacagaagaaaggaaagacaagaactgggaggctgtgataagggagctgcatatatcagcagtgcagcaagtctggctgttgacatggttcttggtgagcccaagagagctgactgctggaaaagagtagaggagaacattttcagcctcagaaatatcactggcctctgatgggagagataagtggtctcagggcctaatgagtgctggagaattcattcattcattcagtgaacatgactgaggcctctcactttgctagacattttggaagacaggggtcaaaatcacagttcctactctcaattagctcacagccctgtactagtgatggacaaagaaccagtatgtgacagttcagactaataagcccaacaagagagggatatacaggacactgtgggacccctaaagggagcaccttgtgcagaggtagaaggataggaatgaacgaggggtgacgggtaacaggaagagagagaagcaccgcaggagtctctgaagagtgttcacagggggtgcgaggcttgctgtgcagaaaccaataggggcaggtgagaaatgctgaccccaagggatgagcaggctcatgtcagggtgctacaaccgtcccctcctcttcactctttcctgcaccccagactccaagtcttaaactaggttatctccccagtggcctggcctgccccccgaatgctctcaaaccagtatcttctaaccctagtcaaaaattaccccttcccttcagctagccattagaattgaaacaaattcccactgccatgtgaaagtctgattatcctactgttcccaaggcaccagccttttagtgggatgtttgctgtagtagattgtatcttccaaaaatggccacaaaatgtttctgagtccacatgctcatccagaaactttctactccctcattaagagatagaatctatttcccttccccttgaaattgggctgcctttgtgacttcttcaataaaaagagctgcttggaacccccacccacagcccttacctcccctgcatccatgagcacacccctctgggactatactgtctaccattgcctccctgacttgggactttggctctggagttcactccctaccccaaggccataaaaaacccccactgcactctttagtccctgggctccagccactgccctctccccagatttctctgttttctgccatctctgtgggatccgcataatctgcctccagcagtttctgggagtgaacccagctatcttgctgaaggtagggtaggggtggatgcaacaatgggctgattgttatcaatatgtatggcaagatattatcttgagatattaatctgtgggtttttctttgctcacttccttgtacagtgaccaaacagcctcacgcaagagtacagttggtaaagagggactgaaaagagccaaaaatgtcaacgttcatatttgtgactctaaaacagcatccaagaatcaaaaaagcaaggcttggggcacaaagcacagagacatgtggaccagggacagggatatacagacagccctatcccagtgcctccagggagaccagagtaaggtgtgctgggccgagggaggggaggagcacatggtgaggagcaggtccacattggaagtcttgggagccccaggagcccctcagctggttgcatattcccagagatgtttgccaagccctgattacatatccacactcccctgaatgaacacaccctccccattccagtgtctaaggactctcatgagccctgcagatctgttaggaacactttcagctctaagcaacaaaagatatgattaacagtgccttaaacactacaggtgtattctttcacacaacaagaaggctgtaagtgggtagtttgttggtaaaaatgcagtttatccaggacctagctcatgagcttaggattcaactagttctggaatcatccttaggaatctataattctgaaaacttcctaggtgattctaatttgcaatcagatatggaagccacttctcccaagtttactaaggctgctgtactctcccctcttctgagttttcggagtccattagctttcagaggagtcaacagtgctaccagtgaacacctgactaatttattcactcaaatggtcagcacaccgtaattgctcgctttttacctggtagcatcagctcagtgagggttgtgaactgggcctagagacatgagaattcagcagcatttccaaactgggtagaatttccacagactatttcaagtgctttttttttttccattcaagaaagatggggcaaccagccaagtaaacatggttgtttttgtctgttttgtgttgctaaaacagaatacctgagactgggtaatttataaacgatgatttatttggctcatgttctggaggctggtgctggaatctggtgagggccttctggctatgccattttctggtggaagcgaaagagagagaaaacagggccaaactcatccttttatcaggaacccactcccacagtaactaacccactcccaagataatggcattaagactgtcctgatgacctcatcacctcttaaaggtcccacctgtcaacactgctgcattgaggattaagtttccaacacatgaaacttgagggacacatttaaaccataacaatggtgggctgaacattgtcttttgcctatattcccacccccaaaattcactacagtatcgagattttgttaaaggcaaaaaacaaataaacaaaccatctcaaggacaaggctaaaagagaaaggagcaagtgtggagagagagaggtaaacacgatgtcggaaaccggaaagcaggtggtaaatgatgagtaacttagagaccaggcacaggttgcagagaggaggcaggaagacaacagactggccccggagcacctggtaggcatagaattggaggccccaggaacctctctggttgtggggtgttggttaaaaggctatactaaatacagcttgatcctttgatcgcttctccactcccatcagacaaggcacctctctcatcctacagaagacataccagagaaggggataagggccaagtcagcatgctgaatggcgagaacagcctgcagcctttcgccactgcatctgagaatcctggtgactcagcttagacacatggggcgacaggctacaaatttcttctctggagaaactgagctcctcaaagaaaagacttataaacaatgactactggggattataatcaaatatacatattcagagaaagccaacacagcacaaaaagcagaataaactttaaggaaaactgtaattaatatcttcggagaaagaatataactgcatctacaaaaaagaacaaactactcataaaacaaaaatgagctctcagttctaaaaaaatataaaaacaggaaaaaaaaatccaatagaatccaaacaggctttactgggaaggtactggaggatatattccacaaaatgaaagagcaaaccaggaaaaaggcatacaaaggattcaagagagagggatccaactaaggagaactgaacgacacatcagagcaggaagccaatgggctccagaggggatgtgttaaaaataaaaaatcagttgattacctgatgtgtttgaactattaagaggagattaacactgctggcaatgcgttggaggagaattagggacagaaaaatatcaaaacaagataattttgaactccagggagaaaaagaagttgtataacaacggaagtattatcagtgtacactgtgtgccttaccggggaaaacatttataataatcacaacagttaactttgagtagttacttaattaaaaaatacaatataattacattggaagaataggggaacaaaagtgctcaatcttcatctttcataggaagaagtcaaagtttctgcctaatctgaaaaatcaacacagaagcatataatttagatacctggggaaacatgtggaactttcaactagccgcgccagttgaaaatgggactggtttctctgatgagaatggctgggtaggaaatggtaatctgtcagaccacaaggaatttttctagtcaacaaactccagatgtttgtgattcttttcctcctggttcactgggttcagccaaagtcctccctagaagattgccaagtgtaagctgagcttgaatctgttccgtgctcccttcttactgatacaacctcgaccagttacttaattctctgtggcacccagtttagtcctcaaacttgtggagattaaacaagattattctcggatcacacaggtcaagcagggctataaaaccgggcagcctggctccaagtctactctctgagccactgtgcaacctacaaacgataacagaaaagaacccaaagacttaacagttagagaaagcccctctgaccccaagcattctctctgttcccctaaccattgttagtcatttctgatttgtccttccagagacagtctgtgtgcacatctttctaaatgcacatctagaaagaagaagcttctgatatcaccttgggcagtcacactcatgcacaaataggagatgtttttatcttttctaataactgatatcaactttgctttccaagtccctatttgggtgcttacactggtgagtgcaggggcaaggacagaggagaaaatagtctcaacgaagggtacctttgcaaaatactccatccaccccagtgtttctgctgtcttctctgatgtgactctcagccatgatgtaggttaaagcgtctatcttagggattccttctccttccccagggtcttttttcctctctccccacaaccctgctctccctcacagccttagagagggcagcagggcttgtggagctcagagacgatgctcaaatgggaacagacaattgtccagcgtggaagcagtcacttctgacctggggtcatggcttggcctggcccctgtggctgacaaggcactactgccatggctgggagttgctggtgaaaggaaatgtcccttctccagctgggtcatcccaaaattggtggactctgaagatatggtagtcccagtgcaggtagcagctgtggtgttcccagattgtttggcttccaccacacccggcactatctccccactgcctcccacctcccacccccagtacgaggcagccttagatctctgtgtttcctgccaatactaactgcctgttggatgaaaatccattaggaattttcaaccaacgttacaaaaccacactcaggctggctttaaccatgaaatagacttactggttctgagtctagagacagggcaggcttcagatgggtcacggtccagtgggttagtaacacccccaagggcctggtttctttccaggcttcatctctgccttccactgagtcgacaccatcctgagcctctttcctgagggaggcaagatggcaccaccagcttctggggcacacacttcctctcacatgcacggtagaggaagggagagcacacactctcagaagagcaagacaacttccctccaagactccaccaaccgcttctcctgacttacttgcccaaatagggtcctgagcctatccctgaacccaccacagtgacactgtctctctccagtcagattgccagaatgaggtgtgttcagcagcactggagagaggtgagcaaaggtgaaaatcagagcagcattagcaggaagaggggacagctgctgggaggccccccgcacacctgcgtccacatgccctcacctgttcttgatgtattctcagggcttggctaagagaacctggggcctgagatgcttgggaactggctcctgggccttcttacattccacaagctggggtggccaaaggtaaccaggatggcagtgtcactatgaccttctttctccgcagccaaccacctggtctcctcatgcccagtcctctcatctgctgcgaagacacatcccaggccctctgggacgggtttgctatagactgaattgtgtccccccagttcatgtgttgaagccctaacctccaatgtgatggtatttggaggtggggcctttgggaggcgattacagttagatgaagtctaaccataattactaatcccatgatgggattagtgtccttataagaagagacacagaggcttgccgcttccctctctgctgtgtgagcatgcagtttcaggccacgtcaggaagaggggcctcggcaggaactgaatcagccagcatcttgatcttggacttcccagcttccaatccatcgaaaacacatttctgttgtttaagccacccagtttgtggtattttgttatggcagaacaagttggttaagacaaggaaaataaacagccaatgcctctcagagccctctctctctgctctctggcctctttatgtagtcaagaggataggaggggggcaagtacagctgttcaggggctgctggatacgtctacctagcatagggcacagaagccaatgctgcaatctgctcagtcagaacttaggtctcttggctcaagacctggtccctatttaaataacagtacttccaagatgagcaatgcagtgagccgtggcagccactgacactacagtacgaatctgctcagcagctccttccctggaagtttcagtgtgaggaaacatgactaggtccgaggcaagaaagagtgtggcgaggcaagactcagagaaagggagacaagctggaactacacaacaagcaagcaaggcaggcaggctctggctacgcagaacgacagcactgtaaagctcctgtggcggtcttccctaccggaggagaaactgattgaagcgcattcggaaacagcacctcatttatttacttatttagaatagacaatatacattatacacacatgaaaaaagcaaccaccacaaaagagagccaatggtgaagagtttctctctcatcctatattggcaattcttataaacctttgcagagacagtttttgcatatttccacatttatgtatgttatttttttctttttaaacaaatagcagcatactacttgccctactctacaccttgctgttaacaacattataccttagagatggttcagtatcacacacacctcaatctacctcttcttcatgactgtacaatattccattctatggaggtactataattagtcaaccatgaaacacaggtgttttcccagcccttaactcttcattgtttaaaaaaaaaaatctgtattcgtgtctattgtgtgccagtcactgttctagggaatagagagtagaaaatgagacattcagtgtcactgccgtggaggagtttacaatccatatgtggaaatgaacatccttgcacatacttctttatgtacatgtgtgaatgtattgttattataaactctcaaggtggaattgctgggtcagagccatgtgcatttctaatttcaatagatattgcaaattgtccaccaaacaggtcatgtcagtttcccctctcaccgtctgtactatcttttcatatgattaaaagtcattatagctttatataccattaggtttcttaaacacaaagtaagttctctaaaatgctcatgataacctgagcaatgactaaggaactagggaacatgacatatcaggacacccttgtggggacacatctgcttctgtgcagaggctggggcagaacctgctggctgatactttcctcacctcctatgtggcacagtcttccagcagccctgggccaggggtgggatatgatgacaggtcttttggagaacgtggtggacagttagcaatgtcactcccccacacagtatgtggcaaggaagaagaatctgtgtacacacaaaatctgtctatgaactgagaaaaaacacagggatacccatgacagaccaaggcctgatttccctcgtattgaaagagcttctacaaatcaaccagaaatccaaccaccccacaggtaagtggacaaagaatatggacagttcttgcaaaggaaatactctgtgttccagaaaatccctgtttataaaataaatactataattaaatgtctacatgcattgctgatcagcatcaatttgcccccattgtaactgttatcactatttaaaatagctaacctcggaagagtgccctgagctcacacagcagcacttggtctcctggtcttttctgtcttccctcttgcttatgactttccatgattctcaccatctcatctcataggcaggaactgcacacacgctgcacaggctgcctgttggccactatcagccattcccacccttcccctcctcgcctcagtgacagaggtggctacttccttcccactaggcattatccctgcagggaccccactggggctctgcagattcccagatccctttctctgagtctgccccttccacttggcatgcttttgcttctgacctaaggctcctgcagctcttctgggagggctgttcttgtgctactgcccttttgtgcccacctatagaaagactgaagtacctgggttatcaacgagggtggctcttagccagtggctgacaggcatagaagaatggaagcccagataccctgcctggggcagggacatctcagaggcattgtttacagttgagagctccccttcaggtcaggctgaacctacctgtcatataactgtctgagatccttgcatggctatccttcttctagctccttactgaattctgctcggagcatttcttttaggaacaatctttgtttctgggcctgcttctaggaaacccaacgtaagacacaatcttcttcctcagtaacaaaatcctgagttttattttggcatatggccaccgtgaataaaaactacatttcccagcttcctttgcaaccaagttcttgccaataagatacagggcacaagtgccctgtgagacttctaggaaatccataaagggagtcctgctgatggctagtgtccatcgtggaccctgagggcaaggggtacatcctcaggatgtgggagcagagatctggaaaaggcctggacctctaacaacctcatggatctgccaataccaaccgcagattgtctaccatcccaccattaccccacaacttcttttgagaaataagttcctctcctgtttaagccaatgtcattcgggtgtttattccatgcagttaaatttaatcctagtttacagaccagaccattgactctgaaaaacgacagacactcagtttgccagcctcccttgcagctaggctttgccagtgtaacccagatctggctgaggaggtataaaggaaggtcttggggggaagaaaggtgtaggcaggaggttctggaaaagatatttcttcctgatgcaaaaaacaaacaggtgcacaatgtccagctctctttccactctggcaacctattccctgctacctgcctttggctgcagcatgtgaagatgtgctgtctggagctgtggcagccattctataaccaggaaactacaagtgcatggacaaaaagccaaccagctgaggatggctgtgcagaaggatggagagagcctgggtctttcagaaactcactgagatctcccactccaaaccaataaatggtccacactgttaatcgggttttccattacatacagttgaaagcaatctaacatactcacagggaacaaagcactgaagtaaaatcacctggaagtgatcaattctcaaaaagcctgctactataacctcttggagggtgctatagtttgggtgtttttgtcccctccaaaattcatgttgaaactcaattcccagtgcaagaatgttgggaggtggggcctagagtgaggtgtttaggtcataagagtgggtactctctcactcttccagcatgtgaggacacagcgttcctccccttcataggatgaagcacgcaaagccccattttggaagcagagacagagctaagaccccaccagacaccaagcctgttggtgcctggatcttggacttccaacctccagaactgtgagaaacagatatctgttctttataaattacccagtctcaggtattctattattgcagcacaaaacaaactatggggagatgactgggttctgggaggtgattacctgtgctaggcttgcctctgagggcaagaaacagcaactccagcttcagggaagtgaaataataagaaataaactccaggatccgctgattcctgtgttcaacaatgccatcaggaacccagggccctcccctctctctgctctgccactcttgaaatgggcttcattctcaggcagccagcaagacagaggcatgcttctgggcagcacagccagacctaactggggcctatcgagggcctgcactctcccccttggcttctccctccagctggattttcttgcttttcttcaaacatgccagataggctcctgccctagcctctgcacttgcgttccctctgcctacagtgcttttgcatacatgtccacttggctctgcctccttcaggtcctcacccaaatattacctcccgagagaggcctgccctgaccacaccttttaagattaaccacctcccaactccccatttctttttctggcttaatttttctccctggcatgtaacttcatccaatatagcacacattcccttggcctcactgagtgtccgggccccacttgcctagaaggtgtgctccaggaaggcagagatgtttaagattgttcaccctcattcccccagggcctggcacaggtgtttcacaattatctccacagtggctgtgccacgaggagccccatcaatgcccgctgcggcctgcccctttctccgccgtcccctttcaccttcgccctgggggcggaggggaggggcccaccacggccttatttccgcgagcgccggcactgcccgctccgagcc

SEQ ID NO: 9233 - RNA, 14222 nt, Homo sapiens
  source 1..14222: mol_type = other RNA
agaccctgcagccttcccacccttccccaggccgctctccccagccctggcctcctgcgttcctcttgtgcagcttctctcgggcacagacacaaacctcaccggagttgtgtgggaagatcccaaagcccttcccaatgccaccctgcagggtactgggatgcatgggggtagttgtggcctgtggtcccactcatgcccctgcttcttgtccctcatgtcacttctttcccaggtgaacatggtccttttttgccttcagtccccaaatccacctgtacaaatttgccagatatggcaggctctccatgaaggttttgggataacacagagggagcacagcgtacccaccaaacagaacaaccttgaggtagaatagggtctgaaggcagggaacctaaggctgtttcacattgacttcatagaactaaattgaaaggaaaaccctaactttccatgcctaagtaacaaaaggaccagaggctactccctttgcaaacccccaccttttctacagggcagatgggaaactgaaagtatctctgattggtgccaagcaaccaatcagatgtttgcataggagtgtaacttcataacttcacttcagcctctgactggttgctgtccacagccaatcagactgattgcggaccaagtcttcctttgcataaaagtgcaactttgtaacttcaccttagcctctcatgctaaagtgaatcttaggagtttgcataggagtgtgacccttgtaaccacttcagcctctgagtggaaagcaaccagattgattgcaggccaccacttcatttacatgggtgaacaccaggtggccagtgggaaacctctaggaggtatttggacccaagaagattgtgtatcaggacccttgtgtccctatgctcgggcccacccccacactgtggacagtactttcattttcaataaatctctgcttttgttgcctcactcttcccttactttgtttgtgtgttttgcccaattctttgttcaagatgccaagaacctggacatgcttcaccaacagcaacctgaaattgaaaaccgctaatcattgttcttaaaaggtccttggccatccaagccctgggggttttctactggcagccctgatctcatactcatcccaccaccagtccctgggtcctccccatccttctgctcttatctccactgcttctcctttcccaggctcttcttccctctccagagctaccctgacatttcagtttcatcttcttttattgtactgtgtgtttcagcaatctgagtgttactgtctcccactcatcctcaccttttgaagaaagaaccaaaaacaaaaacaaaaaaagtcaatataggcctttcaagatactccaaaaacttaagaaaaaagtgttaaggctatattacaagaccccagaaaaatgatgctcagaagacaaaagcagtaatttttagtttaaatagtactttttctctggcagtaagtacatcagggagagtcaagacttcctcttggaaaagtatgccatctggttcttgtcatactgttgtgctccttaactcatttcatgcaaaatttccagcaccatgtttgagggaccctgattactcctcatccatgcagtttcagagccacaggagagatgcatgtgggtgggcagaagtggaagttgtttatgagcatgaagtatttctgagaaatgaacgcattgatgttgggatttgaaatctgatttatctctttgatgattacgggaggaaattttattataaacaataatatttgctggcatatgcatggatgtctgaactcagatgataaaaactagaggattttgagcatcttggaaaaaaattgtacaattaatttaagatttcttacatgacctagaaaatgaaaaggggaagcaaatacactggaaaaaaaagaaggtggaggaggatcacattactccttcacagttaattagaagaactttcaaccaaaacacataactgggtaacaaataccaggtaattttctttgactgaattttttttcacttcattttctttgaagtgaaaaaaagtaatttttaaatacaggaaataatattttatgactgagtattctcttcaaagaatctgggtcagcagctcatttcaaattttcagtgcctagaggacgataatacttagtgctgtttgctggtgatttacaacactttcgtggcttaagaccaagaatatacatattaaaaatcatgctctgcctgaatccaacaagcagatgccccaccttcttttaaggaagaacatgacaataatgaacggataatagagtacaaacaaagacactcaaactgcatttcctaatgttgcaaatgttaatattgagtaacaaagcatcatttctattaaagctggccttcagccactcccttatgaggtaggtggaaagaaatctttttactttcccataattctactacttacgggaaagcaagttgactttgcccagcattgatgcaaagagcatgacacagagttcaagccgcagcactgctgctcaggagagtggaaaagagaaaagttattggcacaatagcaaccaagtgtttcatctaaatgttctgtttcttgagctcccaggtaactcagcttcacatcttttccttgtacaggtcaactccacttaggtagaatgtgaatatatagtatgagaggccaaaaacccatacctatataagcaaaattatctccccctactgccaattcataaaaataacacctgccagaatggaacagaatgctgaaaagtctaccttgaaaagatgagcgattttcaagccaagaaaacttgaatgtatgaaaccccctagaaagaatgtgtcatccagggggtaattggcccatcgcagaaacatggaaaagaggaaaaggaagacagcagggcacagtgttcataagaaagagacacaggatgctttttaagaaacttgggtgtgaaagcaaaacaggcaatatttagaaaggaacttttggtcaatgggtggaaatgggttaaaataggagccatttgcacataattatattctaaggggaaggaagcaatagagagagcaattgaaaatgtaaggaagagagggaagaactgatgtgggtgagggtgcatgtttagaacacaggctgggaagagtcggccgcgggagtcacactgctaataaaaggcagagaccaggggtttttggacctgggtgcaaattgtggtcttgccactttctatctgagggaccttgtcaccctgatggtgaaaaacaagcctgtaacagaagaaaggaaagacaagaactgggaggctgtgataagggagctgcatatatcagcagtgcagcaagtctggctgttgacatggttcttggtgagcccaagagagctgactgctggaaaagagtagaggagaacattttcagcctcagaaatatcactggcctctgatgggagagataagtggtctcagggcctaatgagtgctggagaattcattcattcattcagtgaacatgactgaggcctctcactttgctagacattttggaagacaggggtcaaaatcacagttcctactctcaattagctcacagccctgtactagtgatggacaaagaaccagtatgtgacagttcagactaataagcccaacaagagagggatatacaggacactgtgggacccctaaagggagcaccttgtgcagaggtagaaggataggaatgaacgaggggtgacgggtaacaggaagagagagaagcaccgcaggagtctctgaagagtgttcacagggggtgcgaggcttgctgtgcagaaaccaataggggcaggtgagaaatgctgaccccaagggatgagcaggctcatgtcagggtgctacaaccgtcccctcctcttcactctttcctgcaccccagactccaagtcttaaactaggttatctccccagtggcctggcctgccccccgaatgctctcaaaccagtatcttctaaccctagtcaaaaattaccccttcccttcagctagccattagaattgaaacaaattcccactgccatgtgaaagtctgattatcctactgttcccaaggcaccagccttttagtgggatgtttgctgtagtagattgtatcttccaaaaatggccacaaaatgtttctgagtccacatgctcatccagaaactttctactccctcattaagagatagaatctatttcccttccccttgaaattgggctgcctttgtgacttcttcaataaaaagagctgcttggaacccccacccacagcccttacctcccctgcatccatgagcacacccctctgggactatactgtctaccattgcctccctgacttgggactttggctctggagttcactccctaccccaaggccataaaaaacccccactgcactctttagtccctgggctccagccactgccctctccccagatttctctgttttctgccatctctgtgggatccgcataatctgcctccagcagtttctgggagtgaacccagctatcttgctgaaggtagggtaggggtggatgcaacaatgggctgattgttatcaatatgtatggcaagatattatcttgagatattaatctgtgggtttttctttgctcacttccttgtacagtgaccaaacagcctcacgcaagagtacagttggtaaagagggactgaaaagagccaaaaatgtcaacgttcatatttgtgactctaaaacagcatccaagaatcaaaaaagcaaggcttggggcacaaagcacagagacatgtggaccagggacagggatatacagacagccctatcccagtgcctccagggagaccagagtaaggtgtgctgggccgagggaggggaggagcacatggtgaggagcaggtccacattggaagtcttgggagccccaggagcccctcagctggttgcatattcccagagatgtttgccaagccctgattacatatccacactcccctgaatgaacacaccctccccattccagtgtctaaggactctcatgagccctgcagatctgttaggaacactttcagctctaagcaacaaaagatatgattaacagtgccttaaacactacaggtgtattctttcacacaacaagaaggctgtaagtgggtagtttgttggtaaaaatgcagtttatccaggacctagctcatgagcttaggattcaactagttctggaatcatccttaggaatctataattctgaaaacttcctaggtgattctaatttgcaatcagatatggaagccacttctcccaagtttactaaggctgctgtactctcccctcttctgagttttcggagtccattagctttcagaggagtcaacagtgctaccagtgaacacctgactaatttattcactcaaatggtcagcacaccgtaattgctcgctttttacctggtagcatcagctcagtgagggttgtgaactgggcctagagacatgagaattcagcagcatttccaaactgggtagaatttccacagactatttcaagtgctttttttttttccattcaagaaagatggggcaaccagccaagtaaacatggttgtttttgtctgttttgtgttgctaaaacagaatacctgagactgggtaatttataaacgatgatttatttggctcatgttctggaggctggtgctggaatctggtgagggccttctggctatgccattttctggtggaagcgaaagagagagaaaacagggccaaactcatccttttatcaggaacccactcccacagtaactaacccactcccaagataatggcattaagactgtcctgatgacctcatcacctcttaaaggtcccacctgtcaacactgctgcattgaggattaagtttccaacacatgaaacttgagggacacatttaaaccataacaatggtgggctgaacattgtcttttgcctatattcccacccccaaaattcactacagtatcgagattttgttaaaggcaaaaaacaaataaacaaaccatctcaaggacaaggctaaaagagaaaggagcaagtgtggagagagagaggtaaacacgatgtcggaaaccggaaagcaggtggtaaatgatgagtaacttagagaccaggcacaggttgcagagaggaggcaggaagacaacagactggccccggagcacctggtaggcatagaattggaggccccaggaacctctctggttgtggggtgttggttaaaaggctatactaaatacagcttgatcctttgatcgcttctccactcccatcagacaaggcacctctctcatcctacagaagacataccagagaaggggataagggccaagtcagcatgctgaatggcgagaacagcctgcagcctttcgccactgcatctgagaatcctggtgactcagcttagacacatggggcgacaggctacaaatttcttctctggagaaactgagctcctcaaagaaaagacttataaacaatgactactggggattataatcaaatatacatattcagagaaagccaacacagcacaaaaagcagaataaactttaaggaaaactgtaattaatatcttcggagaaagaatataactgcatctacaaaaaagaacaaactactcataaaacaaaaatgagctctcagttctaaaaaaatataaaaacaggaaaaaaaaatccaatagaatccaaacaggctttactgggaaggtactggaggatatattccacaaaatgaaagagcaaaccaggaaaaaggcatacaaaggattcaagagagagggatccaactaaggagaactgaacgacacatcagagcaggaagccaatgggctccagaggggatgtgttaaaaataaaaaatcagttgattacctgatgtgtttgaactattaagaggagattaacactgctggcaatgcgttggaggagaattagggacagaaaaatatcaaaacaagataattttgaactccagggagaaaaagaagttgtataacaacggaagtattatcagtgtacactgtgtgccttaccggggaaaacatttataataatcacaacagttaactttgagtagttacttaattaaaaaatacaatataattacattggaagaataggggaacaaaagtgctcaatcttcatctttcataggaagaagtcaaagtttctgcctaatctgaaaaatcaacacagaagcatataatttagatacctggggaaacatgtggaactttcaactagccgcgccagttgaaaatgggactggtttctctgatgagaatggctgggtaggaaatggtaatctgtcagaccacaaggaatttttctagtcaacaaactccagatgtttgtgattcttttcctcctggttcactgggttcagccaaagtcctccctagaagattgccaagtgtaagctgagcttgaatctgttccgtgctcccttcttactgatacaacctcgaccagttacttaattctctgtggcacccagtttagtcctcaaacttgtggagattaaacaagattattctcggatcacacaggtcaagcagggctataaaaccgggcagcctggctccaagtctactctctgagccactgtgcaacctacaaacgataacagaaaagaacccaaagacttaacagttagagaaagcccctctgaccccaagcattctctctgttcccctaaccattgttagtcatttctgatttgtccttccagagacagtctgtgtgcacatctttctaaatgcacatctagaaagaagaagcttctgatatcaccttgggcagtcacactcatgcacaaataggagatgtttttatcttttctaataactgatatcaactttgctttccaagtccctatttgggtgcttacactggtgagtgcaggggcaaggacagaggagaaaatagtctcaacgaagggtacctttgcaaaatactccatccaccccagtgtttctgctgtcttctctgatgtgactctcagccatgatgtaggttaaagcgtctatcttagggattccttctccttccccagggtcttttttcctctctccccacaaccctgctctccctcacagccttagagagggcagcagggcttgtggagctcagagacgatgctcaaatgggaacagacaattgtccagcgtggaagcagtcacttctgacctggggtcatggcttggcctggcccctgtggctgacaaggcactactgccatggctgggagttgctggtgaaaggaaatgtcccttctccagctgggtcatcccaaaattggtggactctgaagatatggtagtcccagtgcaggtagcagctgtggtgttcccagattgtttggcttccaccacacccggcactatctccccactgcctcccacctcccacccccagtacgaggcagccttagatctctgtgtttcctgccaatactaactgcctgttggatgaaaatccattaggaattttcaaccaacgttacaaaaccacactcaggctggctttaaccatgaaatagacttactggttctgagtctagagacagggcaggcttcagatgggtcacggtccagtgggttagtaacacccccaagggcctggtttctttccaggcttcatctctgccttccactgagtcgacaccatcctgagcctctttcctgagggaggcaagatggcaccaccagcttctggggcacacacttcctctcacatgcacggtagaggaagggagagcacacactctcagaagagcaagacaacttccctccaagactccaccaaccgcttctcctgacttacttgcccaaatagggtcctgagcctatccctgaacccaccacagtgacactgtctctctccagtcagattgccagaatgaggtgtgttcagcagcactggagagaggtgagcaaaggtgaaaatcagagcagcattagcaggaagaggggacagctgctgggaggccccccgcacacctgcgtccacatgccctcacctgttcttgatgtattctcagggcttggctaagagaacctggggcctgagatgcttgggaactggctcctgggccttcttacattccacaagctggggtggccaaaggtaaccaggatggcagtgtcactatgaccttctttctccgcagccaaccacctggtctcctcatgcccagtcctctcatctgctgcgaagacacatcccaggccctctgggacgggtttgctatagactgaattgtgtccccccagttcatgtgttgaagccctaacctccaatgtgatggtatttggaggtggggcctttgggaggcgattacagttagatgaagtctaaccataattactaatcccatgatgggattagtgtccttataagaagagacacagaggcttgccgcttccctctctgctgtgtgagcatgcagtttcaggccacgtcaggaagaggggcctcggcaggaactgaatcagccagcatcttgatcttggacttcccagcttccaatccatcgaaaacacatttctgttgtttaagccacccagtttgtggtattttgttatggcagaacaagttggttaagacaaggaaaataaacagccaatgcctctcagagccctctctctctgctctctggcctctttatgtagtcaagaggataggaggggggcaagtacagctgttcaggggctgctggatacgtctacctagcatagggcacagaagccaatgctgcaatctgctcagtcagaacttaggtctcttggctcaagacctggtccctatttaaataacagtacttccaagatgagcaatgcagtgagccgtggcagccactgacactacagtacgaatctgctcagcagctccttccctggaagtttcagtgtgaggaaacatgactaggtccgaggcaagaaagagtgtggcgaggcaagactcagagaaagggagacaagctggaactacacaacaagcaagcaaggcaggcaggctctggctacgcagaacgacagcactgtaaagctcctgtggcggtcttccctaccggaggagaaactgattgaagcgcattcggaaacagcacctcatttatttacttatttagaatagacaatatacattatacacacatgaaaaaagcaaccaccacaaaagagagccaatggtgaagagtttctctctcatcctatattggcaattcttataaacctttgcagagacagtttttgcatatttccacatttatgtatgttatttttttctttttaaacaaatagcagcatactacttgccctactctacaccttgctgttaacaacattataccttagagatggttcagtatcacacacacctcaatctacctcttcttcatgactgtacaatattccattctatggaggtactataattagtcaaccatgaaacacaggtgttttcccagcccttaactcttcattgtttaaaaaaaaaaatctgtattcgtgtctattgtgtgccagtcactgttctagggaatagagagtagaaaatgagacattcagtgtcactgccgtggaggagtttacaatccatatgtggaaatgaacatccttgcacatacttctttatgtacatgtgtgaatgtattgttattataaactctcaaggtggaattgctgggtcagagccatgtgcatttctaatttcaatagatattgcaaattgtccaccaaacaggtcatgtcagtttcccctctcaccgtctgtactatcttttcatatgattaaaagtcattatagctttatataccattaggtttcttaaacacaaagtaagttctctaaaatgctcatgataacctgagcaatgactaaggaactagggaacatgacatatcaggacacccttgtggggacacatctgcttctgtgcagaggctggggcagaacctgctggctgatactttcctcacctcctatgtggcacagtcttccagcagccctgggccaggggtgggatatgatgacaggtcttttggagaacgtggtggacagttagcaatgtcactcccccacacagtatgtggcaaggaagaagaatctgtgtacacacaaaatctgtctatgaactgagaaaaaacacagggatacccatgacagaccaaggcctgatttccctcgtattgaaagagcttctacaaatcaaccagaaatccaaccaccccacaggtaagtggacaaagaatatggacagttcttgcaaaggaaatactctgtgttccagaaaatccctgtttataaaataaatactataattaaatgtctacatgcattgctgatcagcatcaatttgcccccattgtaactgttatcactatttaaaatagctaacctcggaagagtgccctgagctcacacagcagcacttggtctcctggtcttttctgtcttccctcttgcttatgactttccatgattctcaccatctcatctcataggcaggaactgcacacacgctgcacaggctgcctgttggccactatcagccattcccacccttcccctcctcgcctcagtgacagaggtggctacttccttcccactaggcattatccctgcagggaccccactggggctctgcagattcccagatccctttctctgagtctgccccttccacttggcatgcttttgcttctgacctaaggctcctgcagctcttctgggagggctgttcttgtgctactgcccttttgtgcccacctatagaaagactgaagtacctgggttatcaacgagggtggctcttagccagtggctgacaggcatagaagaatggaagcccagataccctgcctggggcagggacatctcagaggcattgtttacagttgagagctccccttcaggtcaggctgaacctacctgtcatataactgtctgagatccttgcatggctatccttcttctagctccttactgaattctgctcggagcatttcttttaggaacaatctttgtttctgggcctgcttctaggaaacccaacgtaagacacaatcttcttcctcagtaacaaaatcctgagttttattttggcatatggccaccgtgaataaaaactacatttcccagcttcctttgcaaccaagttcttgccaataagatacagggcacaagtgccctgtgagacttctaggaaatccataaagggagtcctgctgatggctagtgtccatcgtggaccctgagggcaaggggtacatcctcaggatgtgggagcagagatctggaaaaggcctggacctctaacaacctcatggatctgccaataccaaccgcagattgtctaccatcccaccattaccccacaacttcttttgagaaataagttcctctcctgtttaagccaatgtcattcgggtgtttattccatgcagttaaatttaatcctagtttacagaccagaccattgactctgaaaaacgacagacactcagtttgccagcctcccttgcagctaggctttgccagtgtaacccagatctggctgaggaggtataaaggaaggtcttggggggaagaaaggtgtaggcaggaggttctggaaaagatatttcttcctgatgcaaaaaacaaacaggtgcacaatgtccagctctctttccactctggcaacctattccctgctacctgcctttggctgcagcatgtgaagatgtgctgtctggagctgtggcagccattctataaccaggaaactacaagtgcatggacaaaaagccaaccagctgaggatggctgtgcagaaggatggagagagcctgggtctttcagaaactcactgagatctcccactccaaaccaataaatggtccacactgttaatcgggttttccattacatacagttgaaagcaatctaacatactcacagggaacaaagcactgaagtaaaatcacctggaagtgatcaattctcaaaaagcctgctactataacctcttggagggtgctatagtttgggtgtttttgtcccctccaaaattcatgttgaaactcaattcccagtgcaagaatgttgggaggtggggcctagagtgaggtgtttaggtcataagagtgggtactctctcactcttccagcatgtgaggacacagcgttcctccccttcataggatgaagcacgcaaagccccattttggaagcagagacagagctaagaccccaccagacaccaagcctgttggtgcctggatcttggacttccaacctccagaactgtgagaaacagatatctgttctttataaattacccagtctcaggtattctattattgcagcacaaaacaaactatggggagatgactgggttctgggaggtgattacctgtgctaggcttgcctctgagggcaagaaacagcaactccagcttcagggaagtgaaataataagaaataaactccaggatccgctgattcctgtgttcaacaatgccatcaggaacccagggccctcccctctctctgctctgccactcttgaaatgggcttcattctcaggcagccagcaagacagaggcatgcttctgggcagcacagccagacctaactggggcctatcgagggcctgcactctcccccttggcttctccctccagctggattttcttgcttttcttcaaacatgccagataggctcctgccctagcctctgcacttgcgttccctctgcctacagtgcttttgcatacatgtccacttggctctgcctccttcaggtcctcacccaaatattacctcccgagagaggcctgccctgaccacaccttttaagattaaccacctcccaactccccatttctttttctggcttaatttttctccctggcatgtaacttcatccaatatagcacacattcccttggcctcactgagtgtccgggccccacttgcctagaaggtgtgctccaggaaggcagagatgtttaagattgttcaccctcattcccccagggcctggcacaggtgtttcacaattatcttcgccctgggggcggaggggaggggcccaccacggccttatttccgcgagcgccggcactgcccgctccgagcccgtgtctgtcgg

SEQ ID NO: 9234 - RNA, 10854 nt, Homo sapiens
  source 1..10854: mol_type = other RNA
agaccctgcagccttcccacccttccccaggccgctctccccagccctggcctcctgcgttcctcttgtgcagcttctctcgggcacagacacaaacctcaccggagttgtgtgggaagatcccaaagcccttcccaatgccaccctgcagggtactgggatgcatgggggtagttgtggcctgtggtcccactcatgcccctgcttcttgtccctcatgtcacttctttcccaggtgaacatggtccttttttgccttcagtccccaaatccacctgtacaaatttgccagatatggcaggctctccatgaaggttttgggataacacagagggagcacagcgtacccaccaaacagaacaaccttgaggtagaatagggtctgaaggcagggaacctaaggctgtttcacattgacttcatagaactaaattgaaaggaaaaccctaactttccatgcctaagtaacaaaaggaccagaggctactccctttgcaaacccccaccttttctacagggcagatgggaaactgaaagtatctctgattggtgccaagcaaccaatcagatgtttgcataggagtgtaacttcataacttcacttcagcctctgactggttgctgtccacagccaatcagactgattgcggaccaagtcttcctttgcataaaagtgcaactttgtaacttcaccttagcctctcatgctaaagtgaatcttaggagtttgcataggagtgtgacccttgtaaccacttcagcctctgagtggaaagcaaccagattgattgcaggccaccacttcatttacatgggtgaacaccaggtggccagtgggaaacctctaggaggtatttggacccaagaagattgtgtatcaggacccttgtgtccctatgctcgggcccacccccacactgtggacagtactttcattttcaataaatctctgcttttgttgcctcactcttcccttactttgtttgtgtgttttgcccaattctttgttcaagatgccaagaacctggacatgcttcaccaacagcaacctgaaattgaaaaccgctaatcattgttcttaaaaggtccttggccatccaagccctgggggttttctactggcagccctgatctcatactcatcccaccaccagtccctgggtcctccccatccttctgctcttatctccactgcttctcctttcccaggctcttcttccctctccagagctaccctgacatttcagtttcatcttcttttattgtactgtgtgtttcagcaatctgagtgttactgtctcccactcatcctcaccttttgaagaaagaaccaaaaacaaaaacaaaaaaagtcaatataggcctttcaagatactccaaaaacttaagaaaaaagtgttaaggctatattacaagaccccagaaaaatgatgctcagaagacaaaagcagtaatttttagtttaaatagtactttttctctggcagtaagtacatcagggagagtcaagacttcctcttggaaaagtatgccatctggttcttgtcatactgttgtgctccttaactcatttcatgcaaaatttccagcaccatgtttgagggaccctgattactcctcatccatgcagtttcagagccacaggagagatgcatgtgggtgggcagaagtggaagttgtttatgagcatgaagtatttctgagaaatgaacgcattgatgttgggatttgaaatctgatttatctctttgatgattacgggaggaaattttattataaacaataatatttgctggcatatgcatggatgtctgaactcagatgataaaaactagaggattttgagcatcttggaaaaaaattgtacaattaatttaagatttcttacatgacctagaaaatgaaaaggggaagcaaatacactggaaaaaaaagaaggtggaggaggatcacattactccttcacagttaattagaagaactttcaaccaaaacacataactgggtaacaaataccaggtaattttctttgactgaattttttttcacttcattttctttgaagtgaaaaaaagtaatttttaaatacaggaaataatattttatgactgagtattctcttcaaagaatctgggtcagcagctcatttcaaattttcagtgcctagaggacgataatacttagtgctgtttgctggtgatttacaacactttcgtggcttaagaccaagaatatacatattaaaaatcatgctctgcctgaatccaacaagcagatgccccaccttcttttaaggaagaacatgacaataatgaacggataatagagtacaaacaaagacactcaaactgcatttcctaatgttgcaaatgttaatattgagtaacaaagcatcatttctattaaagctggccttcagccactcccttatgaggtaggtggaaagaaatctttttactttcccataattctactacttacgggaaagcaagttgactttgcccagcattgatgcaaagagcatgacacagagttcaagccgcagcactgctgctcaggagagtggaaaagagaaaagttattggcacaatagcaaccaagtgtttcatctaaatgttctgtttcttgagctcccaggtaactcagcttcacatcttttccttgtacaggtcaactccacttaggtagaatgtgaatatatagtatgagaggccaaaaacccatacctatataagcaaaattatctccccctactgccaattcataaaaataacacctgccagaatggaacagaatgctgaaaagtctaccttgaaaagatgagcgattttcaagccaagaaaacttgaatgtatgaaaccccctagaaagaatgtgtcatccagggggtaattggcccatcgcagaaacatggaaaagaggaaaaggaagacagcagggcacagtgttcataagaaagagacacaggatgctttttaagaaacttgggtgtgaaagcaaaacaggcaatatttagaaaggaacttttggtcaatgggtggaaatgggttaaaataggagccatttgcacataattatattctaaggggaaggaagcaatagagagagcaattgaaaatgtaaggaagagagggaagaactgatgtgggtgagggtgcatgtttagaacacaggctgggaagagtcggccgcgggagtcacactgctaataaaaggcagagaccaggggtttttggacctgggtgcaaattgtggtcttgccactttctatctgagggaccttgtcaccctgatggtgaaaaacaagcctgtaacagaagaaaggaaagacaagaactgggaggctgtgataagggagctgcatatatcagcagtgcagcaagtctggctgttgacatggttcttggtgagcccaagagagctgactgctggaaaagagtagaggagaacattttcagcctcagaaatatcactggcctctgatgggagagataagtggtctcagggcctaatgagtgctggagaattcattcattcattcagtgaacatgactgaggcctctcactttgctagacattttggaagacaggggtcaaaatcacagttcctactctcaattagctcacagccctgtactagtgatggacaaagaaccagtatgtgacagttcagactaataagcccaacaagagagggatatacaggacactgtgggacccctaaagggagcaccttgtgcagaggtagaaggataggaatgaacgaggggtgacgggtaacaggaagagagagaagcaccgcaggagtctctgaagagtgttcacagggggtgcgaggcttgctgtgcagaaaccaataggggcaggtgagaaatgctgaccccaagggatgagcaggctcatgtcagggtgctacaaccgtcccctcctcttcactctttcctgcaccccagactccaagtcttaaactaggttatctccccagtggcctggcctgccccccgaatgctctcaaaccagtatcttctaaccctagtcaaaaattaccccttcccttcagctagccattagaattgaaacaaattcccactgccatgtgaaagtctgattatcctactgttcccaaggcaccagccttttagtgggatgtttgctgtagtagattgtatcttccaaaaatggccacaaaatgtttctgagtccacatgctcatccagaaactttctactccctcattaagagatagaatctatttcccttccccttgaaattgggctgcctttgtgacttcttcaataaaaagagctgcttggaacccccacccacagcccttacctcccctgcatccatgagcacacccctctgggactatactgtctaccattgcctccctgacttgggactttggctctggagttcactccctaccccaaggccataaaaaacccccactgcactctttagtccctgggctccagccactgccctctccccagatttctctgttttctgccatctctgtgggatccgcataatctgcctccagcagtttctgggagtgaacccagctatcttgctgaaggtagggtaggggtggatgcaacaatgggctgattgttatcaatatgtatggcaagatattatcttgagatattaatctgtgggtttttctttgctcacttccttgtacagtgaccaaacagcctcacgcaagagtacagttggtaaagagggactgaaaagagccaaaaatgtcaacgttcatatttgtgactctaaaacagcatccaagaatcaaaaaagcaaggcttggggcacaaagcacagagacatgtggaccagggacagggatatacagacagccctatcccagtgcctccagggagaccagagtaaggtgtgctgggccgagggaggggaggagcacatggtgaggagcaggtccacattggaagtcttgggagccccaggagcccctcagctggttgcatattcccagagatgtttgccaagccctgattacatatccacactcccctgaatgaacacaccctccccattccagtgtctaaggactctcatgagccctgcagatctgttaggaacactttcagctctaagcaacaaaagatatgattaacagtgccttaaacactacaggtgtattctttcacacaacaagaaggctgtaagtgggtagtttgttggtaaaaatgcagtttatccaggacctagctcatgagcttaggattcaactagttctggaatcatccttaggaatctataattctgaaaacttcctaggtgattctaatttgcaatcagatatggaagccacttctcccaagtttactaaggctgctgtactctcccctcttctgagttttcggagtccattagctttcagaggagtcaacagtgctaccagtgaacacctgactaatttattcactcaaatggtcagcacaccgtaattgctcgctttttacctggtagcatcagctcagtgagggttgtgaactgggcctagagacatgagaattcagcagcatttccaaactgggtagaatttccacagactatttcaagtgctttttttttttccattcaagaaagatggggcaaccagccaagtaaacatggttgtttttgtctgttttgtgttgctaaaacagaatacctgagactgggtaatttataaacgatgatttatttggctcatgttctggaggctggtgctggaatctggtgagggccttctggctatgccattttctggtggaagcgaaagagagagaaaacagggccaaactcatccttttatcaggaacccactcccacagtaactaacccactcccaagataatggcattaagactgtcctgatgacctcatcacctcttaaaggtcccacctgtcaacactgctgcattgaggattaagtttccaacacatgaaacttgagggacacatttaaaccataacaatggtgggctgaacattgtcttttgcctatattcccacccccaaaattcactacagtatcgagattttgttaaaggcaaaaaacaaataaacaaaccatctcaaggacaaggctaaaagagaaaggagcaagtgtggagagagagaggtaaacacgatgtcggaaaccggaaagcaggtggtaaatgatgagtaacttagagaccaggcacaggttgcagagaggaggcaggaagacaacagactggccccggagcacctggtaggcatagaattggaggccccaggaacctctctggttgtggggtgttggttaaaaggctatactaaatacagcttgatcctttgatcgcttctccactcccatcagacaaggcacctctctcatcctacagaagacataccagagaaggggataagggccaagtcagcatgctgaatggcgagaacagcctgcagcctttcgccactgcatctgagaatcctggtgactcagcttagacacatggggcgacaggctacaaatttcttctctggagaaactgagctcctcaaagaaaagacttataaacaatgactactggggattataatcaaatatacatattcagagaaagccaacacagcacaaaaagcagaataaactttaaggaaaactgtaattaatatcttcggagaaagaatataactgcatctacaaaaaagaacaaactactcataaaacaaaaatgagctctcagttctaaaaaaatataaaaacaggaaaaaaaaatccaatagaatccaaacaggctttactgggaaggtactggaggatatattccacaaaatgaaagagcaaaccaggaaaaaggcatacaaaggattcaagagagagggatccaactaaggagaactgaacgacacatcagagcaggaagccaatgggctccagaggggatgtgttaaaaataaaaaatcagttgattacctgatgtgtttgaactattaagaggagattaacactgctggcaatgcgttggaggagaattagggacagaaaaatatcaaaacaagataattttgaactccagggagaaaaagaagttgtataacaacggaagtattatcagtgtacactgtgtgccttaccggggaaaacatttataataatcacaacagttaactttgagtagttacttaattaaaaaatacaatataattacattggaagaataggggaacaaaagtgctcaatcttcatctttcataggaagaagtcaaagtttctgcctaatctgaaaaatcaacacagaagcatataatttagatacctggggaaacatgtggaactttcaactagccgcgccagttgaaaatgggactggtttctctgatgagaatggctgggtaggaaatggtaatctgtcagaccacaaggaatttttctagtcaacaaactccagatgtttgtgattcttttcctcctggttcactgggttcagccaaagtcctccctagaagattgccaagtgtaagctgagcttgaatctgttccgtgctcccttcttactgatacaacctcgaccagttacttaattctctgtggcacccagtttagtcctcaaacttgtggagattaaacaagattattctcggatcacacaggtcaagcagggctataaaaccgggcagcctggctccaagtctactctctgagccactgtgcaacctcctatgtggcacagtcttccagcagccctgggccaggggtgggatatgatgacaggtcttttggagaacgtggtggacagttagcaatgtcactcccccacacagtatgtggcaaggaagaagaatctgtgtacacacaaaatctgtctatgaactgagaaaaaacacagggatacccatgacagaccaaggcctgatttccctcgtattgaaagagcttctacaaatcaaccagaaatccaaccaccccacaggtaagtggacaaagaatatggacagttcttgcaaaggaaatactctgtgttccagaaaatccctgtttataaaataaatactataattaaatgtctacatgcattgctgatcagcatcaatttgcccccattgtaactgttatcactatttaaaatagctaacctcggaagagtgccctgagctcacacagcagcacttggtctcctggtcttttctgtcttccctcttgcttatgactttccatgattctcaccatctcatctcataggcaggaactgcacacacgctgcacaggctgcctgttggccactatcagccattcccacccttcccctcctcgcctcagtgacagaggtggctacttccttcccactaggcattatccctgcagggaccccactggggctctgcagattcccagatccctttctctgagtctgccccttccacttggcatgcttttgcttctgacctaaggctcctgcagctcttctgggagggctgttcttgtgctactgcccttttgtgcccacctatagaaagactgaagtacctgggttatcaacgagggtggctcttagccagtggctgacaggcatagaagaatggaagcccagataccctgcctggggcagggacatctcagaggcattgtttacagttgagagctccccttcaggtcaggctgaacctacctgtcatataactgtctgagatccttgcatggctatccttcttctagctccttactgaattctgctcggagcatttcttttaggaacaatctttgtttctgggcctgcttctaggaaacccaacgtaagacacaatcttcttcctcagtaacaaaatcctgagttttattttggcatatggccaccgtgaataaaaactacatttcccagcttcctttgcaaccaagttcttgccaataagatacagggcacaagtgccctgtgagacttctaggaaatccataaagggagtcctgctgatggctagtgtccatcgtggaccctgagggcaaggggtacatcctcaggatgtgggagcagagatctggaaaaggcctggacctctaacaacctcatggatctgccaataccaaccgcagattgtctaccatcccaccattaccccacaacttcttttgagaaataagttcctctcctgtttaagccaatgtcattcgggtgtttattccatgcagttaaatttaatcctagtttacagaccagaccattgactctgaaaaacgacagacactcagtttgccagcctcccttgcagctaggctttgccagtgtaacccagatctggctgaggaggtataaaggaaggtcttggggggaagaaaggtgtaggcaggaggttctggaaaagatatttcttcctgatgcaaaaaacaaacaggtgcacaatgtccagctctctttccactctggcaacctattccctgctacctgcctttggctgcagcatgtgaagatgtgctgtctggagctgtggcagccattctataaccaggaaactacaagtgcatggacaaaaagccaaccagctgaggatggctgtgcagaaggatggagagagcctgggtctttcagaaactcactgagatctcccactccaaaccaataaatggtccacactgttaatcgggttttccattacatacagttgaaagcaatctaacatactcacagggaacaaagcactgaagtaaaatcacctggaagtgatcaattctcaaaaagcctgctactataacctcttggagggtgctatagtttgggtgtttttgtcccctccaaaattcatgttgaaactcaattcccagtgcaagaatgttgggaggtggggcctagagtgaggtgtttaggtcataagagtgggtactctctcactcttccagcatgtgaggacacagcgttcctccccttcataggatgaagcacgcaaagccccattttggaagcagagacagagctaagaccccaccagacaccaagcctgttggtgcctggatcttggacttccaacctccagaactgtgagaaacagatatctgttctttataaattacccagtctcaggtattctattattgcagcacaaaacaaactatggggagatgactgggttctgggaggtgattacctgtgctaggcttgcctctgagggcaagaaacagcaactccagcttcagggaagtgaaataataagaaataaactccaggatccgctgattcctgtgttcaacaatgccatcaggaacccagggccctcccctctctctgctctgccactcttgaaatgggcttcattctcaggcagccagcaagacagaggcatgcttctgggcagcacagccagacctaactggggcctatcgagggcctgcactctcccccttggcttctccctccagctggattttcttgcttttcttcaaacatgccagataggctcctgccctagcctctgcacttgcgttccctctgcctacagtgcttttgcatacatgtccacttggctctgcctccttcaggtcctcacccaaatattacctcccgagagaggcctgccctgaccacaccttttaagattaaccacctcccaactccccatttctttttctggcttaatttttctccctggcatgtaacttcatccaatatagcacacattcccttggcctcactgagtgtccgggccccacttgcctagaaggtgtgctccaggaaggcagagatgtttaagattgttcaccctcattcccccagggcctggcacaggtgtttcacaattatcttcgccctgggggcggaggggaggggcccaccacggccttatttccgcgagcgccggcactgcccgctccgagcccgtgtctgtcgg

SEQ ID NO: 9235 - RNA, 7784 nt, Homo sapiens
  source 1..7784: mol_type = other RNA
agaccctgcagccttcccacccttccccaggccgctctccccagccctggcctcctgcgttcctcttgtgcagcttctctcgggcacagacacaaacctcaccggagttgtgtgggaagatcccaaagcccttcccaatgccaccctgcagggtactgggatgcatgggggtagttgtggcctgtggtcccactcatgcccctgcttcttgtccctcatgtcacttctttcccaggtgaacatggtccttttttgccttcagtccccaaatccacctgtacaaatttgccagatatggcaggctctccatgaaggttttgggataacacagagggagcacagcgtacccaccaaacagaacaaccttgaggtagaatagggtctgaaggcagggaacctaaggctgtttcacattgacttcatagaactaaattgaaaggaaaaccctaactttccatgcctaagtaacaaaaggaccagaggctactccctttgcaaacccccaccttttctacagggcagatgggaaactgaaagtatctctgattggtgccaagcaaccaatcagatgtttgcataggagtgtaacttcataacttcacttcagcctctgactggttgctgtccacagccaatcagactgattgcggaccaagtcttcctttgcataaaagtgcaactttgtaacttcaccttagcctctcatgctaaagtgaatcttaggagtttgcataggagtgtgacccttgtaaccacttcagcctctgagtggaaagcaaccagattgattgcaggccaccacttcatttacatgggtgaacaccaggtggccagtgggaaacctctaggaggtatttggacccaagaagattgtgtatcaggacccttgtgtccctatgctcgggcccacccccacactgtggacagtactttcattttcaataaatctctgcttttgttgcctcactcttcccttactttgtttgtgtgttttgcccaattctttgttcaagatgccaagaacctggacatgcttcaccaacagcaacctgaaattgaaaaccgctaatcattgttcttaaaaggtccttggccatccaagccctgggggttttctactggcagccctgatctcatactcatcccaccaccagtccctgggtcctccccatccttctgctcttatctccactgcttctcctttcccaggctcttcttccctctccagagctaccctgacatttcagtttcatcttcttttattgtactgtgtgtttcagcaatctgagtgttactgtctcccactcatcctcaccttttgaagaaagaaccaaaaacaaaaacaaaaaaagtcaatataggcctttcaagatactccaaaaacttaagaaaaaagtgttaaggctatattacaagaccccagaaaaatgatgctcagaagacaaaagcagtaatttttagtttaaatagtactttttctctggcagtaagtacatcagggagagtcaagacttcctcttggaaaagtatgccatctggttcttgtcatactgttgtgctccttaactcatttcatgcaaaatttccagcaccatgtttgagggaccctgattactcctcatccatgcagtttcagagccacaggagagatgcatgtgggtgggcagaagtggaagttgtttatgagcatgaagtatttctgagaaatgaacgcattgatgttgggatttgaaatctgatttatctctttgatgattacgggaggaaattttattataaacaataatatttgctggcatatgcatggatgtctgaactcagatgataaaaactagaggattttgagcatcttggaaaaaaattgtacaattaatttaagatttcttacatgacctagaaaatgaaaaggggaagcaaatacactggaaaaaaaagaaggtggaggaggatcacattactccttcacagttaattagaagaactttcaaccaaaacacataactgggtaacaaataccaggtaattttctttgactgaattttttttcacttcattttctttgaagtgaaaaaaagtaatttttaaatacaggaaataatattttatgactgagtattctcttcaaagaatctgggtcagcagctcatttcaaattttcagtgcctagaggacgataatacttagtgctgtttgctggtgatttacaacactttcgtggcttaagaccaagaatatacatattaaaaatcatgctctgcctgaatccaacaagcagatgccccaccttcttttaaggaagaacatgacaataatgaacggataatagagtacaaacaaagacactcaaactgcatttcctaatgttgcaaatgttaatattgagtaacaaagcatcatttctattaaagctggccttcagccactcccttatgaggtaggtggaaagaaatctttttactttcccataattctactacttacgggaaagcaagttgactttgcccagcattgatgcaaagagcatgacacagagttcaagccgcagcactgctgctcaggagagtggaaaagagaaaagttattggcacaatagcaaccaagtgtttcatctaaatgttctgtttcttgagctcccaggtaactcagcttcacatcttttccttgtacaggtcaactccacttaggtagaatgtgaatatatagtatgagaggccaaaaacccatacctatataagcaaaattatctccccctactgccaattcataaaaataacacctgccagaatggaacagaatgctgaaaagtctaccttgaaaagatgagcgattttcaagccaagaaaacttgaatgtatgaaaccccctagaaagaatgtgtcatccagggggtaattggcccatcgcagaaacatggaaaagaggaaaaggaagacagcagggcacagtgttcataagaaagagacacaggatgctttttaagaaacttgggtgtgaaagcaaaacaggcaatatttagaaaggaacttttggtcaatgggtggaaatgggttaaaataggagccatttgcacataattatattctaaggggaaggaagcaatagagagagcaattgaaaatgtaaggaagagagggaagaactgatgtgggtgagggtgcatgtttagaacacaggctgggaagagtcggccgcgggagtcacactgctaataaaaggcagagaccaggggtttttggacctgggtgcaaattgtggtcttgccactttctatctgagggaccttgtcaccctgatggtgaaaaacaagcctgtaacagaagaaaggaaagacaagaactgggaggctgtgataagggagctgcatatatcagcagtgcagcaagtctggctgttgacatggttcttggtgagcccaagagagctgactgctggaaaagagtagaggagaacattttcagcctcagaaatatcactggcctctgatgggagagataagtggtctcagggcctaatgagtgctggagaattcattcattcattcagtgaacatgactgaggcctctcactttgctagacattttggaagacaggggtcaaaatcacagttcctactctcaattagctcacagccctgtactagtgatggacaaagaaccagtatgtgacagttcagactaataagcccaacaagagagggatatacaggacactgtgggacccctaaagggagcaccttgtgcagaggtagaaggataggaatgaacgaggggtgacgggtaacaggaagagagagaagcaccgcaggagtctctgaagagtgttcacagggggtgcgaggcttgctgtgcagaaaccaataggggcaggtgagaaatgctgaccccaagggatgagcaggctcatgtcagggtgctacaaccgtcccctcctcttcactctttcctgcaccccagactccaagtcttaaactaggttatctccccagtggcctggcctgccccccgaatgctctcaaaccagtatcttctaaccctagtcaaaaattaccccttcccttcagctagccattagaattgaaacaaattcccactgccatgtgaaagtctgattatcctactgttcccaaggcaccagccttttagtgggatgtttgctgtagtagattgtatcttccaaaaatggccacaaaatgtttctgagtccacatgctcatccagaaactttctactccctcattaagagatagaatctatttcccttccccttgaaattgggctgcctttgtgacttcttcaataaaaagagctgcttggaacccccacccacagcccttacctcccctgcatccatgagcacacccctctgggactatactgtctaccattgcctccctgacttgggactttggctctggagttcactccctaccccaaggccataaaaaacccccactgcactctttagtccctgggctccagccactgccctctccccagatttctctgttttctgccatctctgtgggatccgcataatctgcctccagcagtttctgggagtgaacccagctatcttgctgaaggtagggtaggggtggatgcaacaatgggctgattgttatcaatatgtatggcaagatattatcttgagatattaatctgtgggtttttctttgctcacttccttgtacagtgaccaaacagcctcacgcaagagtacagttggtaaagagggactgaaaagagccaaaaatgtcaacgttcatatttgtgactctaaaacagcatccaagaatcaaaaaagcaaggcttggggcacaaagcacagagacatgtggaccagggacagggatatacagacagccctatcccagtgcctccagggagaccagagtaaggtgtgctgggccgagggaggggaggagcacatggtgaggagcaggtccacattggaagtcttgggagccccaggagcccctcagctggttgcatattcccagagatgtttgccaagccctgattacatatccacactcccctgaatgaacacaccctccccattccagtgtctaaggactctcatgagccctgcagatctgttaggaacactttcagctctaagcaacaaaagatatgattaacagtgccttaaacactacaggtgtattctttcacacaacaagaaggctgtaagtgggtagtttgttggtaaaaatgcagtttatccaggacctagctcatgagcttaggattcaactagttctggaatcatccttaggaatctataattctgaaaacttcctaggtgattctaatttgcaatcagatatggaagccacttctcccaagtttactaaggctgctgtactctcccctcttctgagttttcggagtccattagctttcagaggagtcaacagtgctaccagtgaacacctgactaatttattcactcaaatggtcagcacaccgtaattgctcgctttttacctggtagcatcagctcagtgagggttgtgaactgggcctagagacatgagaattcagcagcatttccaaactgggtagaatttccacagactatttcaagtgctttttttttttccattcaagaaagatggggcaaccagccaagtaaacatggttgtttttgtctgttttgtgttgctaaaacagaatacctgagactgggtaatttataaacgatgatttatttggctcatgttctggaggctggtgctggaatctggtgagggccttctggctatgccattttctggtggaagcgaaagagagagaaaacagggccaaactcatccttttatcaggaacccactcccacagtaactaacccactcccaagataatggcattaagactgtcctgatgacctcatcacctcttaaaggtcccacctgtcaacactgctgcattgaggattaagtttccaacacatgaaacttgagggacacatttaaaccataacaatggtgggctgaacattgtcttttgcctatattcccacccccaaaattcactacagtatcgagattttgttaaaggcaaaaaacaaataaacaaaccatctcaaggacaaggctaaaagagaaaggagcaagtgtggagagagagaggtaaacacgatgtcggaaaccggaaagcaggtggtaaatgatgagtaacttagagaccaggcacaggttgcagagaggaggcaggaagacaacagactggccccggagcacctggtaggcatagaattggaggccccaggaacctctctggttgtggggtgttggttaaaaggctatactaaatacagcttgatcctttgatcgcttctccactcccatcagacaaggcacctctctcatcctacagaagacataccagagaaggggataagggccaagtcagcatgctgaatggcgagaacagcctgcagcctttcgccactgcatctgagaatcctggtgactcagcttagacacatggggcgacaggctacaaatttcttctctggagaaactgagctcctcaaagaaaagacttataaacaatgactactggggattataatcaaatatacatattcagagaaagccaacacagcacaaaaagcagaataaactttaaggaaaactgtaattaatatcttcggagaaagaatataactgcatctacaaaaaagaacaaactactcataaaacaaaaatgagctctcagttctaaaaaaatataaaaacaggaaaaaaaaatccaatagaatccaaacaggctttactgggaaggtactggaggatatattccacaaaatgaaagagcaaaccaggaaaaaggcatacaaaggattcaagagagagggatccaactaaggagaactgaacgacacatcagagcaggaagccaatgggctccagaggggatgtgttaaaaataaaaaatcagttgattacctgatgtgtttgaactattaagaggagattaacactgctggcaatgcgttggaggagaattagggacagaaaaatatcaaaacaagataattttgaactccagggagaaaaagaagttgtataacaacggaagtattatcagtgtacactgtgtgccttaccggggaaaacatttataataatcacaacagttaactttgagtagttacttaattaaaaaatacaatataattacattggaagaataggggaacaaaagtgctcaatcttcatctttcataggaagaagtcaaagtttctgcctaatctgaaaaatcaacacagaagcatataatttagatacctggggaaacatgtggaactttcaactagccgcgccagttgaaaatgggactggtttctctgatgagaatggctgggtaggaaatggtaatctgtcagaccacaaggaatttttctagtcaacaaactccagatgtttgtgattcttttcctcctggttcactgggttcagccaaagtcctccctagaagattgccaagtgtaagctgagcttgaatctgttccgtgctcccttcttactgatacaacctcgaccagttacttaattctctgtggcacccagtttagtcctcaaacttgtggagattaaacaagattattctcggatcacacaggtcaagcagggctataaaaccgggcagcctggctccaagtctactctctgagccactgtgcaaccttcgccctgggggcggaggggaggggcccaccacggccttatttccgcgagcgccggcactgcccgctccgagcccgtgtctgtcgg

SEQ ID NO: 9236 - RNA, 13288 nt, Homo sapiens
  source 1..13288: mol_type = other RNA
agaccctgcagccttcccacccttccccaggccgctctccccagccctggcctcctgcgttcctcttgtgcagcttctctcgggcacagacacaaacctcaccggagttgtgtgggaagatcccaaagcccttcccaatgccaccctgcagggtactgggatgcatgggggtagttgtggcctgtggtcccactcatgcccctgcttcttgtccctcatgtcacttctttcccaggtgaacatggtccttttttgccttcagtccccaaatccacctgtacaaatttgccagatatggcaggctctccatgaaggttttgggataacacagagggagcacagcgtacccaccaaacagaacaaccttgaggtagaatagggtctgaaggcagggaacctaaggctgtttcacattgacttcatagaactaaattgaaaggaaaaccctaactttccatgcctaagtaacaaaaggaccagaggctactccctttgcaaacccccaccttttctacagggcagatgggaaactgaaagtatctctgattggtgccaagcaaccaatcagatgtttgcataggagtgtaacttcataacttcacttcagcctctgactggttgctgtccacagccaatcagactgattgcggaccaagtcttcctttgcataaaagtgcaactttgtaacttcaccttagcctctcatgctaaagtgaatcttaggagtttgcataggagtgtgacccttgtaaccacttcagcctctgagtggaaagcaaccagattgattgcaggccaccacttcatttacatgggtgaacaccaggtggccagtgggaaacctctaggaggtatttggacccaagaagattgtgtatcaggacccttgtgtccctatgctcgggcccacccccacactgtggacagtactttcattttcaataaatctctgcttttgttgcctcactcttcccttactttgtttgtgtgttttgcccaattctttgttcaagatgccaagaacctggacatgcttcaccaacagcaacctgaaattgaaaaccgctaatcattgttcttaaaaggtccttggccatccaagccctgggggttttctactggcagccctgatctcatactcatcccaccaccagtccctgggtcctccccatccttctgctcttatctccactgcttctcctttcccaggctcttcttccctctccagagctaccctgacatttcagtttcatcttcttttattgtactgtgtgtttcagcaatctgagtgttactgtctcccactcatcctcaccttttgaagaaagaaccaaaaacaaaaacaaaaaaagtcaatataggcctttcaagatactccaaaaacttaagaaaaaagtgttaaggctatattacaagaccccagaaaaatgatgctcagaagacaaaagcagtaatttttagtttaaatagtactttttctctggcagtaagtacatcagggagagtcaagacttcctcttggaaaagtatgccatctggttcttgtcatactgttgtgctccttaactcatttcatgcaaaatttccagcaccatgtttgagggaccctgattactcctcatccatgcagtttcagagccacaggagagatgcatgtgggtgggcagaagtggaagttgtttatgagcatgaagtatttctgagaaatgaacgcattgatgttgggatttgaaatctgatttatctctttgatgattacgggaggaaattttattataaacaataatatttgctggcatatgcatggatgtctgaactcagatgataaaaactagaggattttgagcatcttggaaaaaaattgtacaattaatttaagatttcttacatgacctagaaaatgaaaaggggaagcaaatacactggaaaaaaaagaaggtggaggaggatcacattactccttcacagttaattagaagaactttcaaccaaaacacataactgggtaacaaataccaggtaattttctttgactgaattttttttcacttcattttctttgaagtgaaaaaaagtaatttttaaatacaggaaataatattttatgactgagtattctcttcaaagaatctgggtcagcagctcatttcaaattttcagtgcctagaggacgataatacttagtgctgtttgctggtgatttacaacactttcgtggcttaagaccaagaatatacatattaaaaatcatgctctgcctgaatccaacaagcagatgccccaccttcttttaaggaagaacatgacaataatgaacggataatagagtacaaacaaagacactcaaactgcatttcctaatgttgcaaatgttaatattgagtaacaaagcatcatttctattaaagctggccttcagccactcccttatgaggtaggtggaaagaaatctttttactttcccataattctactacttacgggaaagcaagttgactttgcccagcattgatgcaaagagcatgacacagagttcaagccgcagcactgctgctcaggagagtggaaaagagaaaagttattggcacaatagcaaccaagtgtttcatctaaatgttctgtttcttgagctcccaggtaactcagcttcacatcttttccttgtacaggtcaactccacttaggtagaatgtgaatatatagtatgagaggccaaaaacccatacctatataagcaaaattatctccccctactgccaattcataaaaataacacctgccagaatggaacagaatgctgaaaagtctaccttgaaaagatgagcgattttcaagccaagaaaacttgaatgtatgaaaccccctagaaagaatgtgtcatccagggggtaattggcccatcgcagaaacatggaaaagaggaaaaggaagacagcagggcacagtgttcataagaaagagacacaggatgctttttaagaaacttgggtgtgaaagcaaaacaggcaatatttagaaaggaacttttggtcaatgggtggaaatgggttaaaataggagccatttgcacataattatattctaaggggaaggaagcaatagagagagcaattgaaaatgtaaggaagagagggaagaactgatgtgggtgagggtgcatgtttagaacacaggctgggaagagtcggccgcgggagtcacactgctaataaaaggcagagaccaggggtttttggacctgggtgcaaattgtggtcttgccactttctatctgagggaccttgtcaccctgatggtgaaaaacaagcctgtaacagaagaaaggaaagacaagaactgggaggctgtgataagggagctgcatatatcagcagtgcagcaagtctggctgttgacatggttcttggtgagcccaagagagctgactgctggaaaagagtagaggagaacattttcagcctcagaaatatcactggcctctgatgggagagataagtggtctcagggcctaatgagtgctggagaattcattcattcattcagtgaacatgactgaggcctctcactttgctagacattttggaagacaggggtcaaaatcacagttcctactctcaattagctcacagccctgtactagtgatggacaaagaaccagtatgtgacagttcagactaataagcccaacaagagagggatatacaggacactgtgggacccctaaagggagcaccttgtgcagaggtagaaggataggaatgaacgaggggtgacgggtaacaggaagagagagaagcaccgcaggagtctctgaagagtgttcacagggggtgcgaggcttgctgtgcagaaaccaataggggcaggtgagaaatgctgaccccaagggatgagcaggctcatgtcagggtgctacaaccgtcccctcctcttcactctttcctgcaccccagactccaagtcttaaactaggttatctccccagtggcctggcctgccccccgaatgctctcaaaccagtatcttctaaccctagtcaaaaattaccccttcccttcagctagccattagaattgaaacaaattcccactgccatgtgaaagtctgattatcctactgttcccaaggcaccagccttttagtgggatgtttgctgtagtagattgtatcttccaaaaatggccacaaaatgtttctgagtccacatgctcatccagaaactttctactccctcattaagagatagaatctatttcccttccccttgaaattgggctgcctttgtgacttcttcaataaaaagagctgcttggaacccccacccacagcccttacctcccctgcatccatgagcacacccctctgggactatactgtctaccattgcctccctgacttgggactttggctctggagttcactccctaccccaaggccataaaaaacccccactgcactctttagtccctgggctccagccactgccctctccccagatttctctgttttctgccatctctgtgggatccgcataatctgcctccagcagtttctgggagtgaacccagctatcttgctgaaggtagggtaggggtggatgcaacaatgggctgattgttatcaatatgtatggcaagatattatcttgagatattaatctgtgggtttttctttgctcacttccttgtacagtgaccaaacagcctcacgcaagagtacagttggtaaagagggactgaaaagagccaaaaatgtcaacgttcatatttgtgactctaaaacagcatccaagaatcaaaaaagcaaggcttggggcacaaagcacagagacatgtggaccagggacagggatatacagacagccctatcccagtgcctccagggagaccagagtaaggtgtgctgggccgagggaggggaggagcacatggtgaggagcaggtccacattggaagtcttgggagccccaggagcccctcagctggttgcatattcccagagatgtttgccaagccctgattacatatccacactcccctgaatgaacacaccctccccattccagtgtctaaggactctcatgagccctgcagatctgttaggaacactttcagctctaagcaacaaaagatatgattaacagtgccttaaacactacaggtgtattctttcacacaacaagaaggctgtaagtgggtagtttgttggtaaaaatgcagtttatccaggacctagctcatgagcttaggattcaactagttctggaatcatccttaggaatctataattctgaaaacttcctaggtgattctaatttgcaatcagatatggaagccacttctcccaagtttactaaggctgctgtactctcccctcttctgagttttcggagtccattagctttcagaggagtcaacagtgctaccagtgaacacctgactaatttattcactcaaatggtcagcacaccgtaattgctcgctttttacctggtagcatcagctcagtgagggttgtgaactgggcctagagacatgagaattcagcagcatttccaaactgggtagaatttccacagactatttcaagtgctttttttttttccattcaagaaagatggggcaaccagccaagtaaacatggttgtttttgtctgttttgtgttgctaaaacagaatacctgagactgggtaatttataaacgatgatttatttggctcatgttctggaggctggtgctggaatctggtgagggccttctggctatgccattttctggtggaagcgaaagagagagaaaacagggccaaactcatccttttatcaggaacccactcccacagtaactaacccactcccaagataatggcattaagactgtcctgatgacctcatcacctcttaaaggtcccacctgtcaacactgctgcattgaggattaagtttccaacacatgaaacttgagggacacatttaaaccataacaatggtgggctgaacattgtcttttgcctatattcccacccccaaaattcactacagtatcgagattttgttaaaggcaaaaaacaaataaacaaaccatctcaaggacaaggctaaaagagaaaggagcaagtgtggagagagagaggtaaacacgatgtcggaaaccggaaagcaggtggtaaatgatgagtaacttagagaccaggcacaggttgcagagaggaggcaggaagacaacagactggccccggagcacctggtaggcatagaattggaggccccaggaacctctctggttgtggggtgttggttaaaaggctatactaaatacagcttgatcctttgatcgcttctccactcccatcagacaaggcacctctctcatcctacagaagacataccagagaaggggataagggccaagtcagcatgctgaatggcgagaacagcctgcagcctttcgccactgcatctgagaatcctggtgactcagcttagacacatggggcgacaggctacaaatttcttctctggagaaactgagctcctcaaagaaaagacttataaacaatgactactggggattataatcaaatatacatattcagagaaagccaacacagcacaaaaagcagaataaactttaaggaaaactgtaattaatatcttcggagaaagaatataactgcatctacaaaaaagaacaaactactcataaaacaaaaatgagctctcagttctaaaaaaatataaaaacaggaaaaaaaaatccaatagaatccaaacaggctttactgggaaggtactggaggatatattccacaaaatgaaagagcaaaccaggaaaaaggcatacaaaggattcaagagagagggatccaactaaggagaactgaacgacacatcagagcaggaagccaatgggctccagaggggatgtgttaaaaataaaaaatcagttgattacctgatgtgtttgaactattaagaggagattaacactgctggcaatgcgttggaggagaattagggacagaaaaatatcaaaacaagataattttgaactccagggagaaaaagaagttgtataacaacggaagtattatcagtgtacactgtgtgccttaccggggaaaacatttataataatcacaacagttaactttgagtagttacttaattaaaaaatacaatataattacattggaagaataggggaacaaaagtgctcaatcttcatctttcataggaagaagtcaaagtttctgcctaatctgaaaaatcaacacagaagcatataatttagatacctggggaaacatgtggaactttcaactagccgcgccagttgaaaatgggactggtttctctgatgagaatggctgggtaggaaatggtaatctgtcagaccacaaggaatttttctagtcaacaaactccagatgtttgtgattcttttcctcctggttcactgggttcagccaaagtcctccctagaagattgccaagtgtaagctgagcttgaatctgttccgtgctcccttcttactgatacaacctcgaccagttacttaattctctgtggcacccagtttagtcctcaaacttgtggagattaaacaagattattctcggatcacacaggtcaagcagggctataaaaccgggcagcctggctccaagtctactctctgagccactgtgcaactggttctgagtctagagacagggcaggcttcagatgggtcacggtccagtgggttagtaacacccccaagggcctggtttctttccaggcttcatctctgccttccactgagtcgacaccatcctgagcctctttcctgagggaggcaagatggcaccaccagcttctggggcacacacttcctctcacatgcacggtagaggaagggagagcacacactctcagaagagcaagacaacttccctccaagactccaccaaccgcttctcctgacttacttgcccaaatagggtcctgagcctatccctgaacccaccacagtgacactgtctctctccagtcagattgccagaatgaggtgtgttcagcagcactggagagaggtgagcaaaggtgaaaatcagagcagcattagcaggaagaggggacagctgctgggaggccccccgcacacctgcgtccacatgccctcacctgttcttgatgtattctcagggcttggctaagagaacctggggcctgagatgcttgggaactggctcctgggccttcttacattccacaagctggggtggccaaaggtaaccaggatggcagtgtcactatgaccttctttctccgcagccaaccacctggtctcctcatgcccagtcctctcatctgctgcgaagacacatcccaggccctctgggacgggtttgctatagactgaattgtgtccccccagttcatgtgttgaagccctaacctccaatgtgatggtatttggaggtggggcctttgggaggcgattacagttagatgaagtctaaccataattactaatcccatgatgggattagtgtccttataagaagagacacagaggcttgccgcttccctctctgctgtgtgagcatgcagtttcaggccacgtcaggaagaggggcctcggcaggaactgaatcagccagcatcttgatcttggacttcccagcttccaatccatcgaaaacacatttctgttgtttaagccacccagtttgtggtattttgttatggcagaacaagttggttaagacaaggaaaataaacagccaatgcctctcagagccctctctctctgctctctggcctctttatgtagtcaagaggataggaggggggcaagtacagctgttcaggggctgctggatacgtctacctagcatagggcacagaagccaatgctgcaatctgctcagtcagaacttaggtctcttggctcaagacctggtccctatttaaataacagtacttccaagatgagcaatgcagtgagccgtggcagccactgacactacagtacgaatctgctcagcagctccttccctggaagtttcagtgtgaggaaacatgactaggtccgaggcaagaaagagtgtggcgaggcaagactcagagaaagggagacaagctggaactacacaacaagcaagcaaggcaggcaggctctggctacgcagaacgacagcactgtaaagctcctgtggcggtcttccctaccggaggagaaactgattgaagcgcattcggaaacagcacctcatttatttacttatttagaatagacaatatacattatacacacatgaaaaaagcaaccaccacaaaagagagccaatggtgaagagtttctctctcatcctatattggcaattcttataaacctttgcagagacagtttttgcatatttccacatttatgtatgttatttttttctttttaaacaaatagcagcatactacttgccctactctacaccttgctgttaacaacattataccttagagatggttcagtatcacacacacctcaatctacctcttcttcatgactgtacaatattccattctatggaggtactataattagtcaaccatgaaacacaggtgttttcccagcccttaactcttcattgtttaaaaaaaaaaatctgtattcgtgtctattgtgtgccagtcactgttctagggaatagagagtagaaaatgagacattcagtgtcactgccgtggaggagtttacaatccatatgtggaaatgaacatccttgcacatacttctttatgtacatgtgtgaatgtattgttattataaactctcaaggtggaattgctgggtcagagccatgtgcatttctaatttcaatagatattgcaaattgtccaccaaacaggtcatgtcagtttcccctctcaccgtctgtactatcttttcatatgattaaaagtcattatagctttatataccattaggtttcttaaacacaaagtaagttctctaaaatgctcatgataacctgagcaatgactaaggaactagggaacatgacatatcaggacacccttgtggggacacatctgcttctgtgcagaggctggggcagaacctgctggctgatactttcctcacctcctatgtggcacagtcttccagcagccctgggccaggggtgggatatgatgacaggtcttttggagaacgtggtggacagttagcaatgtcactcccccacacagtatgtggcaaggaagaagaatctgtgtacacacaaaatctgtctatgaactgagaaaaaacacagggatacccatgacagaccaaggcctgatttccctcgtattgaaagagcttctacaaatcaaccagaaatccaaccaccccacaggtaagtggacaaagaatatggacagttcttgcaaaggaaatactctgtgttccagaaaatccctgtttataaaataaatactataattaaatgtctacatgcattgctgatcagcatcaatttgcccccattgtaactgttatcactatttaaaatagctaacctcggaagagtgccctgagctcacacagcagcacttggtctcctggtcttttctgtcttccctcttgcttatgactttccatgattctcaccatctcatctcataggcaggaactgcacacacgctgcacaggctgcctgttggccactatcagccattcccacccttcccctcctcgcctcagtgacagaggtggctacttccttcccactaggcattatccctgcagggaccccactggggctctgcagattcccagatccctttctctgagtctgccccttccacttggcatgcttttgcttctgacctaaggctcctgcagctcttctgggagggctgttcttgtgctactgcccttttgtgcccacctatagaaagactgaagtacctgggttatcaacgagggtggctcttagccagtggctgacaggcatagaagaatggaagcccagataccctgcctggggcagggacatctcagaggcattgtttacagttgagagctccccttcaggtcaggctgaacctacctgtcatataactgtctgagatccttgcatggctatccttcttctagctccttactgaattctgctcggagcatttcttttaggaacaatctttgtttctgggcctgcttctaggaaacccaacgtaagacacaatcttcttcctcagtaacaaaatcctgagttttattttggcatatggccaccgtgaataaaaactacatttcccagcttcctttgcaaccaagttcttgccaataagatacagggcacaagtgccctgtgagacttctaggaaatccataaagggagtcctgctgatggctagtgtccatcgtggaccctgagggcaaggggtacatcctcaggatgtgggagcagagatctggaaaaggcctggacctctaacaacctcatggatctgccaataccaaccgcagattgtctaccatcccaccattaccccacaacttcttttgagaaataagttcctctcctgtttaagccaatgtcattcgggtgtttattccatgcagttaaatttaatcctagtttacagaccagaccattgactctgaaaaacgacagacactcagtttgccagcctcccttgcagctaggctttgccagtgtaacccagatctggctgaggaggtataaaggaaggtcttggggggaagaaaggtgtaggcaggaggttctggaaaagatatttcttcctgatgcaaaaaacaaacaggtgcacaatgtccagctctctttccactctggcaacctattccctgctacctgcctttggctgcagcatgtgaagatgtgctgtctggagctgtggcagccattctataaccaggaaactacaagtgcatggacaaaaagccaaccagctgaggatggctgtgcagaaggatggagagagcctgggtctttcagaaactcactgagatctcccactccaaaccaataaatggtccacactgttaatcgggttttccattacatacagttgaaagcaatctaacatactcacagggaacaaagcactgaagtaaaatcacctggaagtgatcaattctcaaaaagcctgctactataacctcttggagggtgctatagtttgggtgtttttgtcccctccaaaattcatgttgaaactcaattcccagtgcaagaatgttgggaggtggggcctagagtgaggtgtttaggtcataagagtgggtactctctcactcttccagcatgtgaggacacagcgttcctccccttcataggatgaagcacgcaaagccccattttggaagcagagacagagctaagaccccaccagacaccaagcctgttggtgcctggatcttggacttccaacctccagaactgtgagaaacagatatctgttctttataaattacccagtctcaggtattctattattgcagcacaaaacaaactatggggagatgactgggttctgggaggtgattacctgtgctaggcttgcctctgagggcaagaaacagcaactccagcttcagggaagtgaaataataagaaataaactccaggatccgctgattcctgtgttcaacaatgccatcaggaacccagggccctcccctctctctgctctgccactcttgaaatgggcttcattctcaggcagccagcaagacagaggcatgcttctgggcagcacagccagacctaactggggcctatcgagggcctgcactctcccccttggcttctccctccagctggattttcttgcttttcttcaaacatgccagataggctcctgccctagcctctgcacttgcgttccctctgcctacagtgcttttgcatacatgtccacttggctctgcctccttcaggtcctcacccaaatattacctcccgagagaggcctgccctgaccacaccttttaagattaaccacctcccaactccccatttctttttctggcttaatttttctccctggcatgtaacttcatccaatatagcacacattcccttggcctcactgagtgtccgggccccacttgcctagaaggtgtgctccaggaaggcagagatgtttaagattgttcaccctcattcccccagggcctggcacaggtgtttcacaattatcttcgccctgggggcggaggggaggggcccaccacggccttatttccgcgagcgccggcactgcccgctccgagcccgtgtctgtcgg

SEQ ID NO: 9237 - RNA, 2027 nt, Homo sapiens
  source 1..2027: mol_type = other RNA
agacctggcccagacctcagctacacaagctgatggactgagtcaggggccacactctccctcctctggtgatgtgacctcagctggtttcttcccactcggccatgggtttcccatcctggagtgggattaagaatccttgtcctggccctgtgcagtggccacacctgtaatcccgacactttgggaagcttagatgggagaatccctaggggccaggagttcaataccagcctgggcaacatagggagaccctgtctctacaaaaaaaatttttaacaattagcccggtgtggtggtgtgagcctgtagtcctagctacttagaggcagatgtgggaggatcacttgagcccagtttgaggctagtccaggcaacatggcaagatcctatctctaccaaaaatatatataaacgtgcgtgtgtgtgtgtgtgtgtgtgtgtgtataaatatataaaagaatccttgtcctgcctgtctcatgggcagcttggaggaaacactgtttttttgttttttttttttttgagatggagttttgctcttgttgcccaggctggagtgcaatggcacgatctcagctcaactgcaacctccacctcctgggtttaagcgattttcctgcctcatcctcccgagtagctgagattacaggtgcccaccaccacacctggctaattttttgcatttttagtagagatggggtttcaccatgttggccaggatggtctcgaactcctgacctcaggtgagccaccccactcggcctcccgaagtgctgggattacaggcatgagccactgcgcccagcctggaaacactattgacaagtgaggaggcctagtccattgagtatcagctagggctacaaacttccaaatcggtgaatcaggtccagagagggacaagtgccccagggttacacaatcatttgctgaagcagaggttgctgccatctttggcctcacccaactggaccacttccttgggcactgagtgacatagctccagcaggtctggattctgcagcttggtccttatcttctggctcagggtcagctccgggctcggcctgtgctgctgcagggcctccaggaccgagcgggccttctcaaagggggggatcttcagccggtacaggatctctgcccgcagatagttgccaatgccattgaagaacctctggtccaggagggcctcgcagatgggccggtcaaaggccttatccgctaggtttcgtagcacattctccctggaggaacacggtctgggtgcgtaagacccatccccaccctccatgggatggggagaggggctcagagaacctgtttctgagccctggaggttaaggctgcaatgagctgtgatggcgccactgtactctagcctaggcaacagagcgagaccctgaactgctggtactcctgcaagacacagggcccgcggcccggctgccactttcccccaaggtcccagcggccgaaccggcggatgtccacgaaacatagggcgagccgggggccaggcggggccgtgtaaaagcgcaggtgggcatggcgtggcagctcctcgcggggcaccagctgaaaagagccggacatgccgaagcggaagaccagggccagtggctcctgttggggctgggccccaggcagagggctcagtatcaggcgcagctccttgccgcgggctgaagctgagatgcggtaggcactgctctcaaagggcacctcagggttgcggctgacagaggacttctccacgcagccgccgaacaccagcgccctgcaggcctcattcacaaactggctggccaggtgcagctcggggccctcaggcatcctgagggagggtggcagagtcccggacaggtgcctggaaagcccagggcgctgggagctggggctgcagagggagcaggactctgccttgctgctaaccgcttccttccatgggcttccaccgcgtttagacgaaagtcccaatccttgcggggccgcggctgcagccttacttcttcccggct

SEQ ID NO: 9238 - RNA, 2363 nt, Homo sapiens
  source 1..2363: mol_type = other RNA
agacctggcccagacctcagctacacaagctgatggactgagtcaggggccacactctccctcctctggtgatgtgacctcagctggtttcttcccactcggccatgggtttcccatcctggagtgggattaagaatccttgtcctggccctgtgcagtggccacacctgtaatcccgacactttgggaagcttagatgggagaatccctaggggccaggagttcaataccagcctgggcaacatagggagaccctgtctctacaaaaaaaatttttaacaattagcccggtgtggtggtgtgagcctgtagtcctagctacttagaggcagatgtgggaggatcacttgagcccagtttgaggctagtccaggcaacatggcaagatcctatctctaccaaaaatatatataaacgtgcgtgtgtgtgtgtgtgtgtgtgtgtgtataaatatataaaagaatccttgtcctgcctgtctcatgggcagcttggaggaaacactgtttttttgttttttttttttttgagatggagttttgctcttgttgcccaggctggagtgcaatggcacgatctcagctcaactgcaacctccacctcctgggtttaagcgattttcctgcctcatcctcccgagtagctgagattacaggtgcccaccaccacacctggctaattttttgcatttttagtagagatggggtttcaccatgttggccaggatggtctcgaactcctgacctcaggtgagccaccccactcggcctcccgaagtgctgggattacaggcatgagccactgcgcccagcctggaaacactattgacaagtgaggaggcctagtccattgagtatcagctagggctacaaacttccaaatcggtgaatcaggtccagagagggacaagtgccccagggttacacaatcatttgctgaagcagaggttgctgccatctttggcctcacccaactggaccacttccttgggcactgagtgacatagctccagcaggtctggattctgcagcttggtccttatcttctggctcagggtcagctccgggctcggcctgtgctgctgcagggcctccaggaccgagcgggccttctcaaagggggggatcttcagccggtacaggatctctgcccgcagatagttgccaatgccattgaagaacctctggtccaggagggcctcgcagatgggccggtcaaaggccttatccgctaggtttcgtagcacattctccctggaggaacacggtctgggtgcgtaagacccatccccaccctccatgggatggggagaggggctcagagaacctgtttctgagccctggaggttaaggctgcaatgagctgtgatggcgccactgtactctagcctaggcaacagagcgagaccctgaactgctggtactcctgcaagacacagggcccgcggcccggctgccactttcccccaaggtcccagcggccgaaccggcggatgtccacgaaacatagggcgagccgggggccaggcggggccgtgtaaaagcgcaggtgggcatggcgtggcagctcctcgcggggcaccagctgaaaagagccggacatgccgaagcggaagaccagggccagtggctcctgttggggctgggccccaggcagagggctcagtatcaggcgcagctccttgccgcgggctgaagctgagatgcggtaggcactgctctcaaagggcacctcagggttgcggctgacagaggacttctccacgcagccgccgaacaccagcgccctgcaggcctcattcacaaactggctggccaggtgcagctcggggccctcaggcatcctgagggagggtggcagagtcctccgccctccctgctttgccacttgcctctgtccccgggcggttcggaatcggaggcgaaggtgtgcctggctgggaggtggcggaagaacctgacttcccactgcctggcgccggcgagatgcgggggcaggtctgaggccccgggtcgccgctgtctctgcggttgggggaagtcacccagctagcgtgggacagggtcggcacccccagcaggaaacagcagcgacgagccagagcggagtcgcctgcagctgcgcgcaggacgtgcacaggtgcgcggtacgcacaggccctagggacccggtggggatcttaagcaccaacgaacagtcagacctaactcataaacaaacatcatcacggcctgccctgtcagaagcgcagccaagcaacaacaacaacaaaaaaaggcgaggaggtagacccacttgagatggttctgttgcggagagtctctgaaatcagaaagcgccagtccgcaaaaacgaggaaaccc

SEQ ID NO: 9239 - RNA, 2031 nt, Homo sapiens
  source 1..2031: mol_type = other RNA
agacctggcccagacctcagctacacaagctgatggactgagtcaggggccacactctccctcctctggtgatgtgacctcagctggtttcttcccactcggccatgggtttcccatcctggagtgggattaagaatccttgtcctggccctgtgcagtggccacacctgtaatcccgacactttgggaagcttagatgggagaatccctaggggccaggagttcaataccagcctgggcaacatagggagaccctgtctctacaaaaaaaatttttaacaattagcccggtgtggtggtgtgagcctgtagtcctagctacttagaggcagatgtgggaggatcacttgagcccagtttgaggctagtccaggcaacatggcaagatcctatctctaccaaaaatatatataaacgtgcgtgtgtgtgtgtgtgtgtgtgtgtgtataaatatataaaagaatccttgtcctgcctgtctcatgggcagcttggaggaaacactgtttttttgttttttttttttttgagatggagttttgctcttgttgcccaggctggagtgcaatggcacgatctcagctcaactgcaacctccacctcctgggtttaagcgattttcctgcctcatcctcccgagtagctgagattacaggtgcccaccaccacacctggctaattttttgcatttttagtagagatggggtttcaccatgttggccaggatggtctcgaactcctgacctcaggtgagccaccccactcggcctcccgaagtgctgggattacaggcatgagccactgcgcccagcctggaaacactattgacaagtgaggaggcctagtccattgagtatcagctagggctacaaacttccaaatcggtgaatcaggtccagagagggacaagtgccccagggttacacaatcatttgctgaagcagaggttgctgccatctttggcctcacccaactggaccacttccttgggcactgagtgacatagctccagcaggtctggattctgcagcttggtccttatcttctggctcagggtcagctccgggctcggcctgtgctgctgcagggcctccaggaccgagcgggccttctcaaagggggggatcttcagccggtacaggatctctgcccgcagatagttgccaatgccattgaagaacctctggtccaggagggcctcgcagatgggccggtcaaaggccttatccgctaggtttcgtagcacattctccctggaggaacacggtctgggtgcgtaagacccatccccaccctccatgggatggggagaggggctcagagaacctgtttctgagccctggaggttaaggctgcaatgagctgtgatggcgccactgtactctagcctaggcaacagagcgagaccctgaactgctggtactcctgcaagacacagggcccgcggcccggctgccactttcccccaaggtcccagcggccgaaccggcggatgtccacgaaacatagggcgagccgggggccaggcggggccgtgtaaaagcgcaggtgggcatggcgtggcagctcctcgcggggcaccagctgaaaagagccggacatgccgaagcggaagaccagggccagtggctcctgttggggctgggccccaggcagagggctcagtatcaggcgcagctccttgccgcgggctgaagctgagatgcggtaggcactgctctcaaagggcacctcagggttgcggctgacagaggacttctccacgcagccgccgaacaccagcgccctgcaggcctcattcacaaactggctggccaggtgcagctcggggccctcaggcatcctgagggagggtggcagagtcctccgccctccctgctttgccacttgcctctgtccccgggcggttcggaatcggaggcgaaggtgtgccttaagtggaagggggcacttagcgacggcagacgcccgtaccttgccccctccacacctgggagccgcccctggcctggcacccacagggctcgtttt

SEQ ID NO: 9240 - RNA, 2004 nt, Homo sapiens
  source 1..2004: mol_type = other RNA
agacctggcccagacctcagctacacaagctgatggactgagtcaggggccacactctccctcctctggtgatgtgacctcagctggtttcttcccactcggccatgggtttcccatcctggagtgggattaagaatccttgtcctggccctgtgcagtggccacacctgtaatcccgacactttgggaagcttagatgggagaatccctaggggccaggagttcaataccagcctgggcaacatagggagaccctgtctctacaaaaaaaatttttaacaattagcccggtgtggtggtgtgagcctgtagtcctagctacttagaggcagatgtgggaggatcacttgagcccagtttgaggctagtccaggcaacatggcaagatcctatctctaccaaaaatatatataaacgtgcgtgtgtgtgtgtgtgtgtgtgtgtgtataaatatataaaagaatccttgtcctgcctgtctcatgggcagcttggaggaaacactgtttttttgttttttttttttttgagatggagttttgctcttgttgcccaggctggagtgcaatggcacgatctcagctcaactgcaacctccacctcctgggtttaagcgattttcctgcctcatcctcccgagtagctgagattacaggtgcccaccaccacacctggctaattttttgcatttttagtagagatggggtttcaccatgttggccaggatggtctcgaactcctgacctcaggtgagccaccccactcggcctcccgaagtgctgggattacaggcatgagccactgcgcccagcctggaaacactattgacaagtgaggaggcctagtccattgagtatcagctagggctacaaacttccaaatcggtgaatcaggtccagagagggacaagtgccccagggttacacaatcatttgctgaagcagaggttgctgccatctttggcctcacccaactggaccacttccttgggcactgagtgacatagctccagcaggtctggattctgcagcttggtccttatcttctggctcagggtcagctccgggctcggcctgtgctgctgcagggcctccaggaccgagcgggccttctcaaagggggggatcttcagccggtacaggatctctgcccgcagatagttgccaatgccattgaagaacctctggtccaggagggcctcgcagatgggccggtcaaaggccttatccgctaggtttcgtagcacattctccctggaggaacacggtctgggtgcgtaagacccatccccaccctccatgggatggggagaggggctcagagaacctgtttctgagccctggaggttaaggctgcaatgagctgtgatggcgccactgtactctagcctaggcaacagagcgagaccctgaactgctggtactcctgcaagacacagggcccgcggcccggctgccactttcccccaaggtcccagcggccgaaccggcggatgtccacgaaacatagggcgagccgggggccaggcggggccgtgtaaaagcgcaggtgggcatggcgtggcagctcctcgcggggcaccagctgaaaagagccggacatgccgaagcggaagaccagggccagtggctcctgttggggctgggccccaggcagagggctcagtatcaggcgcagctccttgccgcgggctgaagctgagatgcggtaggcactgctctcaaagggcacctcagggttgcggctgacagaggacttctccacgcagccgccgaacaccagcgccctgcaggcctcattcacaaactggctggccaggtgcagctcggggccctcaggcatcctgagggagggtggcagagtcctctgtccccgggcggttcggaatcggaggcgaaggtgtgccttaagtggaagggggcacttagcgacggcagacgcccgtaccttgccccctccacacctgggagccgcccctggcctggcacccacagggctcgtttt

SEQ ID NO: 9241 - RNA, 263 nt, Homo sapiens
  source 1..263: mol_type = other RNA
agactgaccttcaaccccacagatccttccagccctgggggtgttgaatccagtcatcttccacccagatctactctagggtggctggcacaaagatctcccctacacctggcccaggctgagggcagatgactcatgaagcccccttccaccttctgcctttggcctctgatcccacttcctccagaatcagttctgagatggctgccctctgctcccgaaactccctcaggcacctgagtcacccgcaggctttggcttct

SEQ ID NO: 9242 - RNA, 143 nt, Homo sapiens
  source 1..143: mol_type = other RNA
agactgacggctggaggcccattctgcctgggccccgggcattgggtccagcaccaccgcccccacctccacggcccaggctggcgctgggcgtgctgccacagctgctgctgatgacctgcagctgccgctcggcacggtca

SEQ ID NO: 9243 - RNA, 81 nt, Homo sapiens
  source 1..81: mol_type = other RNA
agagaagaagatcagcctgcatttagcagtccacatctgcaggctgatcttcttctcttttggattctatctcttgctgct

SEQ ID NO: 9244 - RNA, 1333 nt, Homo sapiens
  source 1..1333: mol_type = other RNA
agagattggtagaaatcaggtgacagctccctggccacagctctcgcgatgtcgcactcctggcgagcggccagcgcggcctggtcggcggcatcggccttcgctctggcatgtgcagtccttgaatttgctatttccactttggttctggccatggcagctgccctttgggcgccttcaattgctctgtccaccttctccctagtttttgtatgtcttattggtataagctgcttccttatcccacggaccagaatattatttttgtattttccctcttctttggagccgtcaggaaacacggtacagccatatccatgcctcttgttatttgcccactccccttcatacttcatgccattggagcgctcgctaacgccgaagccgttgcgcttgtcgttcttccactcgcccatgtaggtttccgtggtggtggcgtccacgtggtcttccaccgggcaaaaatcacaatctacatcgccaaagctgatcgtggagttggcatcgctggaactaattctgctcatggccgcgtcgctgcggacagagctgcgcttgctcgagatggaagacttggattcggacttgcgaagtttcatgcttccaagaagggagcccctccggaagaggccgcccttcttcttgcccgctagctcagcgtctgcgtggaagttgagcacgaaaccgccgcgggtgccggccgggctgtcggcggcggctgcggcgtcgtggagcacgctgccattgctctgctcgctgcgcagcgaggccagcgaggtacgcagcggtgagcggatcaccgtggccatgccgtagggcacgctctggcgcacgccgtagccatgccgcatgcctccggcccactggccctggtaggtacctccgtccccgtaggtctccacgccgtacccgtcttgcagcccgttactccaggtaccctcgtagcgagcgggggtgcacaggctctgccggaccccgtagcgccccttgaaaccatgtgaccactccccccggtacatccacttgcccttcgtctccacccccagcccgtgccgcttgccctgcgcccagtagccctggtaggtgttgccgctgggccaggtgtagcctccgaccacctcgaagccgtgcgaccaggagcccgagtactcgccctggcccttgggccccgtgcagatgccatgcccgtgcgccttgccctcctcccagccgccgcagtaggtgccgccatcgtcgaagtcgaaccttccgcccgtcattcggggggcagccccggcgcgctccccgcaggggcacggacgcgggcagtgctgggcacggcagggtgtagctc

SEQ ID NO: 9245 - RNA, 1512 nt, Homo sapiens
  source 1..1512: mol_type = other RNA
agagattggtagaaatcaggtgacagctccctggccacagctctcgcgatgtcgcactcctggcgagcggccagcgcggcctggtcggcggcatcggccttcgctctggcatgtgcagtccttgaatttgctatttccactttggttctggccatggcagctgccctttgggcgccttcaattgctctgtccaccttctccctagtttttgtatgtcttattggtataagctgcttccttatcccacggaccagaatattatttttgtattttccctcttctttggagccgtcaggaaacacggtacagccatatccatgcctcttgttatttgcccactccccttcatacttcatgccattggagcgctcgctaacgccgaagccgttgcgcttgtcgttcttccactcgcccatgtaggtttccgtggtggtggcgtccacgtggtcttccaccgggcaaaaatcacaatctacatcgccaaagctgatcgtggagttggcatcgctggaactaattctgctcatggccgcgtcgctgcggacagagctgcgcttgctcgagatggaagacttggattcggacttgcgaagtttcatgcttccaagaagggagcccctccggaagaggccgcccttcttcttgcccgctagctcagcgtctgcgtggaagttgagcacgaaaccgccgcgggtgccggccgggctgtcggcggcggctgcggcgtcgtggagcacgctgccattgctctgctcgctgcgcagcgaggccagcgaggtacgcagcggtgagcggatcaccgtggccatgccgtagggcacgctctggcgcacgccgtagccatgccgcatgcctccggcccactggccctggtaggtacctccgtccccgtaggtctccacgccgtacccgtcttgcagcccgttactccaggtaccctcgtagcgagcgggggtgcacaggctctgccggaccccgtagcgccccttgaaaccatgtgaccactccccccggtacatccacttgcccttcgtctccacccccagcccgtgccgcttgccctgcgcccagtagccctggtaggtgttgccgctgggccaggtgtagcctccgaccacctcgaagccgtgcgaccaggagcccgagtactcgccctggcccttgggccccgtgcagatgccatgcccgtgcgccttgccctcctcccagccgccgcagtaggtgccgccatcgtcgaagtcgaaccttccgcccgtcattcggggggcagccccggcgcgctccccgcaggggcacggacgcgggcagtgctgggcacggcagggtgtagctcgggggtgggggcccggcgggcgagctcacgacagcgccctgggcagctcgcgctgccgctcggctccagtccgacgccgcccccgtcctccctcctcttttgccgccgccaccgccgccttcctcctcctcctcctcctccttcgccgccgccgcctgggccagcgccgcgcgcgagag

SEQ ID NO: 9246 - RNA, 48 nt, Homo sapiens
  source 1..48: mol_type = other RNA
agagattggtagaaatcaggtgagagggtcaagtcataagctggctga

SEQ ID NO: 9247 - RNA, 30 nt, Homo sapiens
  source 1..30: mol_type = other RNA
agagctgagactagaaagcccagggcaggt

SEQ ID NO: 9248 - RNA, 32 nt, Homo sapiens
  source 1..32: mol_type = other RNA
agagctgagactagaaagcccagggcaggtcc

SEQ ID NO: 9249 - RNA, 284 nt, Homo sapiens
  source 1..284: mol_type = other RNA
agagctggctgaagggcagcaaggagggtgcagagccacagcaagaggcccgaagtaataagcttttctccctcactagaacctcccacccccaatccacttaacaatttgtgttctcactctggaatcatcaaagcataagaaatctgctattggaacaggaaatgccaagatagcacaagctctttttttttttttttttttttttccccaaatgtcccatcttttctaatctgggcttttgaagcagagccccttggcagggggagagaaagcacaatcca

SEQ ID NO: 9250 - RNA, 546 nt, Homo sapiens
  source 1..546: mol_type = other RNA
agagctggctgaagggcagcaggaccgggtggccgttgaccaggacggagcccttggtcagctggatgaccacgccatccaccttcatgaggaccctgctcagcgtgggggccgctgactcctggctgcggcgtagctggatgttaaaatcctcgtaggcggcaccgcagtgctcggagaacacgtagttgcagaggccggggaagcggaagacgtcgccgtcgaaggtcttgtagtggaagctgccccaggtgctgcacacccgcccgttgtgcgccgggttggaggctcgtaccacagggatggtcctcagagatgggaagacagtcgccccacggagcgggaccccgctgggcccccgggcgataggagagagggcagggtggtgcttgtagctggattcggaggagccatcctgggcatggcctgtatgccgggtgcaggccagagcgagagccagggcccagagcagggccagcttcctccggccaacactcattgtgtggacggcggggaagagtgccctgtccctcagcagcctctgag

SEQ ID NO: 9251 - RNA, 2055 nt, Homo sapiens
  source 1..2055: mol_type = other RNA
agagctggctgaagggcaggccaccaagatggggaacttcacattcacgggagggaaactggggccctccgggaggctaatcaggactgatgagtatcctgaaaccagtggcaggaatgcacattccagggcttgttctagaagcttatctgtgattaaacagcaggccttgagtcacattacttcatttttttttttctgttgcacactgcaaatggaaagttctggattccacctagggcaccatcgggaggccaatggggtcatatggagacacacgcagatcctgcagcaaagcttctaggttgttcctcagcatggcgtagggcggcttctcctcatacgtgagggccatcaccaccttcaggtacttctgcagggtctctgagggcctgatccagtgaccgcagggtcccacgaagggccccggcttatcaacaaacactggtcagggagctcgtggctgtgaggggccaatgggcggtatccaaacattttgaggagattttaactggtaggttcaaagcaagcaggctcgacttcaggaggtcatgctgtgcctgagagggggtcactgtggcatccgcacagttcagtggaatgtgggggccagcggggccgtcaagtaggctgtctgtggctgactcaaagggagggaggtggtcccccggaggcggctgcataacggagatatctgggtcaaccacacggaggaactgggaggaggtggaaaactgcaaactgctgacggtgaccgagccttgtttctggcatgacaaagtccagcttacattaaaatgaatcccaaggcaacttctgtttttgcttcatgatgtcctcagtgttgggaaggcaatttgtccatggcagaaacccgtagagccacttcagcatgcagtagcccaggctctggaggtcgctgcggcgggagggcccgcatcccttgtgcaggtccatgctaatgaactcaaggtccccctcgtgagggctcctgctgccttccacgtaggccacgtgtttgccacttgggcaatagcggaaggcgaagccatagcctgccaaagtcacctgactctggtcctctggatccacaaagatattttcagctgtcacatttccatgaacatactcattctcatggaggaactccagggcatccagcagccggcaggccacctgcagcacagacctctctgacagcacatgctttgggctgacatccagggccgactgaaggctcctccccaggctgggtaacaccaagaacctgtatttgtcctggtgaacaccgaaacccatgcaggtagggatggccagcagtggggtcgagtacagcttcttccacttgttgacagtttgagtgagaacttttgcttctgtggtcctgagtcacaggtgagggtggaggtgggtgcagcttcatagagaatgccctggttgtccctggtctggaaggacttcagcttccactgtcgcccactcttgtctgtcagcactgtccctgtgggcaaagcttcaagtgaggtggtcactcggctccgcttcagcgtctgagggctctgcctggtcttctgagggctacagctggtcttctgagggctacccctggtcacctgagggctcttcctggtcttctgagggctgcttttgggggttgggggtctgctcccggagcctttggatctctcagaggaactcagagtatcttcagactcagaactgtcaccatctgagaagagggataatcggggagaggtgacggtgctggaccatttcactttcttaggagaggtttcaaaactggagttcagccctctctttgagccttggaaggatgacacatgtggattgacaaaggtctgggaccctacatgctcctctacaggcaaagaatttccacagtaggggcagaatttgaatgccgcttggatacttttgccacagtctggacagaaggagatcatgctttatgaggtcacggtctggcccttggatttactgggttggaaactccatcttgacagcgaccttctcagttgcccagcgaaaacttcc

SEQ ID NO: 9252 - RNA, 2135 nt, Homo sapiens
  source 1..2135: mol_type = other RNA
agagctggctgaagggcaggccaccaagatggggaacttcacattcacgggagggaaactggggccctccgggaggctaatcaggactgatgagtatcctgaaaccagtggcaggaatgcacattccagggcttgttctagaagcttatctgtgattaaacagcaggccttgagtcacattacttcatttttttttttctgttgcacactgcaaatggaaagttctggattccacctagggcaccatcgggaggccaatggggtcatatggagacacacgcagatcctgcagcaaagcttctaggttgttcctcagcatggcgtagggcggcttctcctcatacgtgagggccatcaccaccttcaggtacttctgcagggtctctgagggcctgatccagtgaccgcagggtcccacgaagggccccggcttatcaacaaacactggtcagggagctcgtggctgtgaggggccaatgggcggtatccaaacattttgaggagattttaactggtaggttcaaagcaagcaggctcgacttcaggaggtcatgctgtgcctgagagggggtcactgtggcatccgcacagttcagtggaatgtgggggccagcggggccgtcaagtaggctgtctgtggctgactcaaagggagggaggtggtcccccggaggcggctgcataacggagatatctgggtcaaccacacggaggaactgggaggaggtggaaaactgcaaactgctgacggtgaccgagccttgtttctggcatgacaaagtccagcttacattaaaatgaatcccaaggcaacttctgtttttgcttcatgatgtcctcagtgttgggaaggcaatttgtccatggcagaaacccgtagagccacttcagcatgcagtagcccaggctctggaggtcgctgcggcgggagggcccgcatcccttgtgcaggtccatgctaatgaactcaaggtccccctcgtgagggctcctgctgccttccacgtaggccacgtgtttgccacttgggcaatagcggaaggcgaagccatagcctgccaaagtcacctgactctggtcctctggatccacaaagatattttcagctgtcacatttccatgaacatactcattctcatggaggaactccagggcatccagcagccggcaggccacctgcagcacagacctctctgacagcacatgctttgggctgacatccagggccgactgaaggctcctccccaggctgggtaacaccaagaacctgtatttgtcctggtgaacaccgaaacccatgcaggtagggatggccagcagtggggtcgagtacagcttcttccacttgttgacttgcagaggcttggcggcccgctggaagaagttctgctcattgaacaagcgcccatccttggcatccagtttgagtgagaacttttgcttctgtggtcctgagtcacaggtgagggtggaggtgggtgcagcttcatagagaatgccctggttgtccctggtctggaaggacttcagcttccactgtcgcccactcttgtctgtcagcactgtccctgtgggcaaagcttcaagtgaggtggtcactcggctccgcttcagcgtctgagggctctgcctggtcttctgagggctacagctggtcttctgagggctacccctggtcacctgagggctcttcctggtcttctgagggctgcttttgggggttgggggtctgctcccggagccttggaaggatgacacatgtggattgacaaaggtctgggaccctacatgctcctctacaggcaaagaatttccacagtaggggcagaatttgaatgccgcttggatacttttgccacagtctggacagaaggagatcatgctttatgaggtcacggtctggcccttggatttactgggttggaaactccatcttgacagcgaccttctcagttgcccagcgaaaacttccgctgggcggagagcgctgcgcgcgcatcctgaatctgaggcgcccgcgcaggcgccgctgacttcctgacggcccctgggcttcgcctgcctgggaactccgtttcccagatgcctccgcggcaggcccgccctctgattccagacggaatggggattattcc

SEQ ID NO: 9253 - RNA, 2212 nt, Homo sapiens
  source 1..2212: mol_type = other RNA
agagctggctgaagggcaggccaccaagatggggaacttcacattcacgggagggaaactggggccctccgggaggctaatcaggactgatgagtatcctgaaaccagtggcaggaatgcacattccagggcttgttctagaagcttatctgtgattaaacagcaggccttgagtcacattacttcatttttttttttctgttgcacactgcaaatggaaagttctggattccacctagggcaccatcgggaggccaatggggtcatatggagacacacgcagatcctgcagcaaagcttctaggttgttcctcagcatggcgtagggcggcttctcctcatacgtgagggccatcaccaccttcaggtacttctgcagggtctctgagggcctgatccagtgaccgcagggtcccacgaagggccccggcttatcaacaaacactggtcagggagctcgtggctgtgaggggccaatgggcggtatccaaacattttgaggagattttaactggtaggttcaaagcaagcaggctcgacttcaggaggtcatgctgtgcctgagagggggtcactgtggcatccgcacagttcagtggaatgtgggggccagcggggccgtcaagtaggctgtctgtggctgactcaaagggagggaggtggtcccccggaggcggctgcataacggagatatctgggtcaaccacacggaggaactgggaggaggtggaaaactgcaaactgctgacggtgaccgagccttgtttctggcatgacaaagtccagcttacattaaaatgaatcccaaggcaacttctgtttttgcttcatgatgtcctcagtgttgggaaggcaatttgtccatggcagaaacccgtagagccacttcagcatgcagtagcccaggctctggaggtcgctgcggcgggagggcccgcatcccttgtgcaggtccatgctaatgaactcaaggtccccctcgtgagggctcctgctgccttccacgtaggccacgtgtttgccacttgggcaatagcggaaggcgaagccatagcctgccaaagtcacctgactctggtcctctggatccacaaagatattttcagctgtcacatttccatgaacatactcattctcatggaggaactccagggcatccagcagccggcaggccacctgcagcacagacctctctgacagcacatgctttgggctgacatccagggccgactgaaggctcctccccaggctgggtaacaccaagaacctgtatttgtcctggtgaacaccgaaacccatgcaggtagggatggccagcagtggggtcgagtacagcttcttccacttgttgacttgcagaggcttggcggcccgctggaagaagttctgctcattgaacaagcgcccatccttggcatccagtttgagtgagaacttttgcttctgtggtcctgagtcacaggtgagggtggaggtgggtgcagcttcatagagaatgccctggttgtccctggtctggaaggacttcagcttccactgtcgcccactcttgtctgtcagcactgtccctgtgggcaaagcttcaagtgaggtggtcactcggctccgcttcagcgtctgagggctctgcctggtcttctgagggctacagctggtcttctgagggctacccctggtcacctgagggctcttcctggtcttctgagggctgcttttgggggttgggggtctgctcccggagcctttggatctctcagaggaactcagagtatcttcagactcagaactgtcaccatctgagaagagggataatcggggagaggtgacggtgctggaccatttcactttcttaggagaggtttcaaaactggagttcagccctctctttgagccttggaaggatgacacatgtggattgacaaaggtctgggaccctacatgctcctctacaggcaaagaatttccacagtaggggcagaatttgaatgccgcttggatacttttgccacagtctggacagaaggagatcatgctttatgaggtcacggtctggcccttggatttactgggttggaaactccatcttgacagcgacctctgtacttggggactggggtgggattctgggcttctgcagcctgaccctcggatcctccgcagttacccggactcaccttctcagttgcccagcgaaaacttccgctgggcggag

SEQ ID NO: 9254 - RNA, 2122 nt, Homo sapiens
  source 1..2122: mol_type = other RNA
agagctggctgaagggcaggccaccaagatggggaacttcacattcacgggagggaaactggggccctccgggaggctaatcaggactgatgagtatcctgaaaccagtggcaggaatgcacattccagggcttgttctagaagcttatctgtgattaaacagcaggccttgagtcacattacttcatttttttttttctgttgcacactgcaaatggaaagttctggattccacctagggcaccatcgggaggccaatggggtcatatggagacacacgcagatcctgcagcaaagcttctaggttgttcctcagcatggcgtagggcggcttctcctcatacgtgagggccatcaccaccttcaggtacttctgcagggtctctgagggcctgatccagtgaccgcagggtcccacgaagggccccggcttatcaacaaacactggtcagggagctcgtggctgtgaggggccaatgggcggtatccaaacattttgaggagattttaactggtaggttcaaagcaagcaggctcgacttcaggaggtcatgctgtgcctgagagggggtcactgtggcatccgcacagttcagtggaatgtgggggccagcggggccgtcaagtaggctgtctgtggctgactcaaagggagggaggtggtcccccggaggcggctgcataacggagatatctgggtcaaccacacggaggaactgggaggaggtggaaaactgcaaactgctgacggtgaccgagccttgtttctggcatgacaaagtccagcttacattaaaatgaatcccaaggcaacttctgtttttgcttcatgatgtcctcagtgttgggaaggcaatttgtccatggcagaaacccgtagagccacttcagcatgcagtagcccaggctctggaggtcgctgcggcgggagggcccgcatcccttgtgcaggtccatgctaatgaactcaaggtccccctcgtgagggctcctgctgccttccacgtaggccacgtgtttgccacttgggcaatagcggaaggcgaagccatagcctgccaaagtcacctgactctggtcctctggatccacaaagatattttcagctgtcacatttccatgaacatactcattctcatggaggaactccagggcatccagcagccggcaggccacctgcagcacagacctctctgacagcacatgctttgggctgacatccagggccgactgaaggctcctccccaggctgggtaacaccaagaacctgtatttgtcctggtgaacaccgaaacccatgcaggtagggatggccagcagtggggtcgagtacagcttcttccacttgttgacttgcagaggcttggcggcccgctggaagaagttctgctcattgaacaagcgcccatccttggcatccagtttgagtgagaacttttgcttctgtggtcctgagtcacaggtgagggtggaggtgggtgcagcttcatagagaatgccctggttgtccctggtctggaaggacttcagcttccactgtcgcccactcttgtctgtcagcactgtccctgtgggcaaagcttcaagtgaggtggtcactcggctccgcttcagcgtctgagggctctgcctggtcttctgagggctacagctggtcttctgagggctacccctggtcacctgagggctcttcctggtcttctgagggctgcttttgggggttgggggtctgctcccggagcctttggatctctcagaggaactcagagtatcttcagactcagaactgtcaccatctgagaagagggataatcggggagaggtgacggtgctggaccatttcactttcttaggagaggtttcaaaactggagttcagccctctctttgagccttggaaggatgacacatgtggattgacaaaggtctgggaccctacatgctcctctacaggcaaagaatttccacagtaggggcagaatttgaatgccgcttggatacttttgccacagtctggacagaaggagatcatgctttatgaggtcacggtctggcccttggatttactgggttggaaactccatcttgacagcgaccttctcagttgcccagcgaaaacttcc

SEQ ID NO: 9255 - RNA, 2926 nt, Homo sapiens
  source 1..2926: mol_type = other RNA
agagctggctgaagggcaggccaccaagatggggaacttcacattcacgggagggaaactggggccctccgggaggctaatcaggactgatgagtatcctgaaaccagtggcaggaatgcacattccagggcttgttctagaagcttatctgtgattaaacagcaggccttgagtcacattacttcatttttttttttctgttgcacactgcaaatggaaagttctggattccacctagggcaccatcgggaggccaatggggtcatatggagacacacgcagatcctgcagcaaagcttctaggttgttcctcagcatggcgtagggcggcttctcctcatacgtgagggccatcaccaccttcaggtacttctgcagggtctctgagggcctgatccagtgaccgcagggtcccacgaagggccccggcttatcaacaaacctgaagggacagaaacacatgtgaaaggtctcttagggaaaggagagcaaccttttaaaacagaatgcctaagatatatacacagcctaagatatatacacagtcccctctgccatccagggaagttatgttcttaaagtcactgtgaacactgaatcaaccaatccactaccattgctcccaagggaaacagcactgcttcctgcaagcctctggccacacgattttccccgatcaatacaccttgttttggccgggcacagtggctcacgcctgtaatcccaacactttgggaggccgaggggggtggatcacgaggtcaggagatccgagatcatcctggctaacacggtgaaactgtccctactaaaaatataaaaaactagccgggtgtggtggcgggtgcctgtggtcccagctactcgggaggctgaggcaggagaatggcatgaatctgggaggcagagcttgcagtgagcctagattgagccactgcactccagcctgggcgacagagagagactccgtctcaaaaacaaaacaaaacaaaacaatacaccttgttttatgtatgtttctgttgaaatacatcttatgtaataagtattgttgattcattagcattgaactcttttaatctgtgatccttaagacggagaggatccctttgatgatgaggaaagatccaagatggaaataaagattttattacttacaggtcctgggggcacaccgcacacccaaaggtgacctccccacccgtcccaagcacacacacagacacacacacacacacacacgcacactggtcagggagctcgtggctgtgaggggccaatgggcggtatccaaacattttgaggagattttaactggtaggttcaaagcaagcaggctcgacttcaggaggtcatgctgtgcctgagagggggtcactgtggcatccgcacagttcagtggaatgtgggggccagcggggccgtcaagtaggctgtctgtggctgactcaaagggagggaggtggtcccccggaggcggctgcataacggagatatctgggtcaaccacacggaggaactgggaggaggtggaaaactgcaaactgctgacggtgaccgagccttgtttctggcatgacaaagtccagcttacattaaaatgaatcccaaggcaacttctgtttttgcttcatgatgtcctcagtgttgggaaggcaatttgtccatggcagaaacccgtagagccacttcagcatgcagtagcccaggctctggaggtcgctgcggcgggagggcccgcatcccttgtgcaggtccatgctaatgaactcaaggtccccctcgtgagggctcctgctgccttccacgtaggccacgtgtttgccacttgggcaatagcggaaggcgaagccatagcctgccaaagtcacctgactctggtcctctggatccacaaagatattttcagctgtcacatttccatgaacatactcattctcatggaggaactccagggcatccagcagccggcaggccacctgcagcacagacctctctgacagcacatgctttgggctgacatccagggccgactgaaggctcctccccaggctgggtaacaccaagaacctgtatttgtcctggtgaacaccgaaacccatgcaggtagggatggccagcagtggggtcgagtacagcttcttccacttgttgacttgcagaggcttggcggcccgctggaagaagttctgctcattgaacaagcgcccatccttggcatccagtttgagtgagaacttttgcttctgtggtcctgagtcacaggtgagggtggaggtgggtgcagcttcatagagaatgccctggttgtccctggtctggaaggacttcagcttccactgtcgcccactcttgtctgtcagcactgtccctgtgggcaaagcttcaagtgaggtggtcactcggctccgcttcagcgtctgagggctctgcctggtcttctgagggctacagctggtcttctgagggctacccctggtcacctgagggctcttcctggtcttctgagggctgcttttgggggttgggggtctgctcccggagcctttggatctctcagaggaactcagagtatcttcagactcagaactgtcaccatctgagaagagggataatcggggagaggtgacggtgctggaccatttcactttcttaggagaggtttcaaaactggagttcagccctctctttgagccttggaaggatgacacatgtggattgacaaaggtctgggaccctacatgctcctctacaggcaaagaatttccacagtaggggcagaatttgaatgccgcttggatacttttgccacagtctggacagaaggagatcatgctttatgaggtcacggtctggcccttggatttactgggttggaaactccatcttgacagcgaccttctcagttgcccagcgaaaacttcc

SEQ ID NO: 9256 - RNA, 1799 nt, Homo sapiens
  source 1..1799: mol_type = other RNA
agagctggctgaagggcaggccaccaagatggggaacttcacattcacgggagggaaactggggccctccgggaggctaatcaggactgatgagtatcctgaaaccagtggcaggaatgcacattccagggcttgttctagaagcttatctgtgattaaacagcaggccttgagtcacattacttcatttttttttttctgttgcacactgcaaatggaaagttctggattccacctagggcaccatcgggaggccaatggggtcatatggagacacacgcagatcctgcagcaaagcttctaggttgttcctcagcatggcgtagggcggcttctcctcatacgtgagggccatcaccaccttcaggtacttctgcagggtctctgagggcctgatccagtgaccgcagggtcccacgaagggccccggcttatcaacaaacttctgtttttgcttcatgatgtcctcagtgttgggaaggcaatttgtccatggcagaaacccgtagagccacttcagcatgcagtagcccaggctctggaggtcgctgcggcgggagggcccgcatcccttgtgcaggtccatgctaatgaactcaaggtccccctcgtgagggctcctgctgccttccacgtaggccacgtgtttgccacttgggcaatagcggaaggcgaagccatagcctgccaaagtcacctgactctggtcctctggatccacaaagatattttcagctgtcacatttccatgaacatactcattctcatggaggaactccagggcatccagcagccggcaggccacctgcagcacagacctctctgacagcacatgctttgggctgacatccagggccgactgaaggctcctccccaggctgggtaacaccaagaacctgtatttgtcctggtgaacaccgaaacccatgcaggtagggatggccagcagtggggtcgagtacagcttcttccacttgttgacttgcagaggcttggcggcccgctggaagaagttctgctcattgaacaagcgcccatccttggcatccagtttgagtgagaacttttgcttctgtggtcctgagtcacaggtgagggtggaggtgggtgcagcttcatagagaatgccctggttgtccctggtctggaaggacttcagcttccactgtcgcccactcttgtctgtcagcactgtccctgtgggcaaagcttcaagtgaggtggtcactcggctccgcttcagcgtctgagggctctgcctggtcttctgagggctacagctggtcttctgagggctacccctggtcacctgagggctcttcctggtcttctgagggctgcttttgggggttgggggtctgctcccggagccttggaaggatgacacatgtggattgacaaaggtctgggaccctacatgctcctctacaggcaaagaatttccacagtaggggcagaatttgaatgccgcttggatacttttgccacagtctggacagaaggagatcatgctttatgaggtcacggtctggcccttggatttactgggttggaaactccatcttgacagcgacctcagcgcaggtggggcgattgcctaggcgacgacagagcctcccttcggccgcacctccatagaaaccacgggatgacttagacgccaagtttcacagcggaggagctgtcgaacttcccacaagttccgcccatctccgccttagccatgcccaacacggagcccaaggtggcttgggaagctcaagaggaggccagtgaaccccgcgacccggagccgctct

SEQ ID NO: 9257 - RNA, 1680 nt, Homo sapiens
  source 1..1680: mol_type = other RNA
agagctggctgaagggcaggccaccaagatggggaacttcacattcacgggagggaaactggggccctccgggaggctaatcaggactgatgagtatcctgaaaccagtggcaggaatgcacattccagggcttgttctagaagcttatctgtgattaaacagcaggccttgagtcacattacttcatttttttttttctgttgcacactgcaaatggaaagttctggattccacctagggcaccatcgggaggccaatggggtcatatggagacacacgcagatcctgcagcaaagcttctaggttgttcctcagcatggcgtagggcggcttctcctcatacgtgagggccatcaccaccttcaggtacttctgcagggtctctgagggcctgatccagtgaccgcagggtcccacgaagggccccggcttatcaacaaacttctgtttttgcttcatgatgtcctcagtgttgggaaggcaatttgtccatggcagaaacccgtagagccacttcagcatgcagtagcccaggctctggaggtcgctgcggcgggagggcccgcatcccttgtgcaggtccatgctaatgaactcaaggtccccctcgtgagggctcctgctgccttccacgtaggccacgtgtttgccacttgggcaatagcggaaggcgaagccatagcctgccaaagtcacctgactctggtcctctggatccacaaagatattttcagctgtcacatttccatgaacatactcattctcatggaggaactccagggcatccagcagccggcaggccacctgcagcacagacctctctgacagcacatgctttgggctgacatccagggccgactgaaggctcctccccaggctgggtaacaccaagaacctgtatttgtcctggtgaacaccgaaacccatgcaggtagggatggccagcagtggggtcgagtacagcttcttccacttgttgacttgcagaggcttggcggcccgctggaagaagttctgctcattgaacaagcgcccatccttggcatccagtttgagtgagaacttttgcttctgtggtcctgagtcacaggtgagggtggaggtgggtgcagcttcatagagaatgccctggttgtccctggtctggaaggacttcagcttccactgtcgcccactcttgtctgtcagcactgtccctgtgggcaaagcttcaagtgaggtggtcactcggctccgcttcagcgtctgagggctctgcctggtcttctgagggctacagctggtcttctgagggctacccctggtcacctgagggctcttcctggtcttctgagggctgcttttgggggttgggggtctgctcccggagccttggaaggatgacacatgtggattgacaaaggtctgggaccctacatgctcctctacaggcaaagaatttccacagtaggggcagaatttgaatgccgcttggatacttttgccacagtctggacagaaggagatcatgctttatgaggtcacggtctggcccttggatttactgggttggaaactccatcttgacagcgacctctgtacttggggactggggtgggattctgggcttctgcagcctgaccctcggatcctccgcagttacccggactcaccttctcagttgcccagcgaaaacttcc

SEQ ID NO: 9258 - RNA, 1764 nt, Homo sapiens
  source 1..1764: mol_type = other RNA
agagctggctgaagggcaggccaccaagatggggaacttcacattcacgggagggaaactggggccctccgggaggctaatcaggactgatgagtatcctgaaaccagtggcaggaatgcacattccagggcttgttctagaagcttatctgtgattaaacagcaggccttgagtcacattacttcatttttttttttctgttgcacactgcaaatggaaagttctggattccacctagggcaccatcgggaggccaatggggtcatatggagacacacgcagatcctgcagcaaagcttctaggttgttcctcagcatggcgtagggcggcttctcctcatacgtgagggccatcaccaccttcaggtacttctgcagggtctctgagggcctgatccagtgaccgcagggtcccacgaagggccccggcttatcaacaaacttctgtttttgcttcatgatgtcctcagtgttgggaaggcaatttgtccatggcagaaacccgtagagccacttcagcatgcagtagcccaggctctggaggtcgctgcggcgggagggcccgcatcccttgtgcaggtccatgctaatgaactcaaggtccccctcgtgagggctcctgctgccttccacgtaggccacgtgtttgccacttgggcaatagcggaaggcgaagccatagcctgccaaagtcacctgactctggtcctctggatccacaaagatattttcagctgtcacatttccatgaacatactcattctcatggaggaactccagggcatccagcagccggcaggccacctgcagcacagacctctctgacagcacatgctttgggctgacatccagggccgactgaaggctcctccccaggctgggtaacaccaagaacctgtatttgtcctggtgaacaccgaaacccatgcaggtagggatggccagcagtggggtcgagtacagcttcttccacttgttgacttgcagaggcttggcggcccgctggaagaagttctgctcattgaacaagcgcccatccttggcatccagtttgagtgagaacttttgcttctgtggtcctgagtcacaggtgagggtggaggtgggtgcagcttcatagagaatgccctggttgtccctggtctggaaggacttcagcttccactgtcgcccactcttgtctgtcagcactgtccctgtgggcaaagcttcaagtgaggtggtcactcggctccgcttcagcgtctgagggctctgcctggtcttctgagggctacagctggtcttctgagggctacccctggtcacctgagggctcttcctggtcttctgagggctgcttttgggggttgggggtctgctcccggagccttggaaggatgacacatgtggattgacaaaggtctgggaccctacatgctcctctacaggcaaagaatttccacagtaggggcagaatttgaatgccgcttggatacttttgccacagtctggacagaaggagatcatgctttatgaggtcacggtctggcccttggatttactgggttggaaactccatcttgacagcgaccttctcagttgcccagcgaaaacttccgctgggcggagagcgctgcgcgcgcatcctgaatctgaggcgcccgcgcaggcgccgctgacttcctgacggcccctgggcttcgcctgcctgggaactccgtttcccagatgcctccgcggcaggcccgccctctgattccagacggaatggggattattcc

SEQ ID NO: 9259 - RNA, 2147 nt, Homo sapiens
  source 1..2147: mol_type = other RNA
agagctggctgaagggcaggccaccaagatggggaacttcacattcacgggagggaaactggggccctccgggaggctaatcaggactgatgagtatcctgaaaccagtggcaggaatgcacattccagggcttgttctagaagcttatctgtgattaaacagcaggccttgagtcacattacttcatttttttttttctgttgcacactgcaaatggaaagttctggattccacctagggcaccatcgggaggccaatggggtcatatggagacacacgcagatcctgcagcaaagcttctaggttgttcctcagcatggcgtagggcggcttctcctcatacgtgagggccatcaccaccttcaggtacttctgcagggtctctgagggcctgatccagtgaccgcagggtcccacgaagggccccggcttatcaacaaacttctgtttttgcttcatgatgtcctcagtgttgggaaggcaatttgtccatggcagaaacccgtagagccacttcagcatgcagtagcccaggctctggaggtcgctgcggcgggagggcccgcatcccttgtgcaggtccatgctaatgaactcaaggtccccctcgtgagggctcctgctgccttccacgtaggccacgtgtttgccacttgggcaatagcggaaggcgaagccatagcctgccaaagtcacctgactctggtcctctggatccacaaagatattttcagctgtcacatttccatgaacatactcattctcatggaggaactccagggcatccagcagccggcaggccacctgcagcacagacctctctgacagcacatgctttgggctgacatccagggccgactgaaggctcctccccaggctgggtaacaccaagaacctgtatttgtcctggtgaacaccgaaacccatgcaggtagggatggccagcagtggggtcgagtacagcttcttccacttgttgacttgcagaggcttggcggcccgctggaagaagttctgctcattgaacaagcgcccatccttggcatccagtttgagtgagaacttttgcttctgtggtcctgagtcacaggtgagggtggaggtgggtgcagcttcatagagaatgccctggttgtccctggtctggaaggacttcagcttccactgtcgcccactcttgtctgtcagcactgtccctgtgggcaaagcttcaagtgaggtggtcactcggctccgcttcagcgtctgagggctctgcctggtcttctgagggctacagctggtcttctgagggctacccctggtcacctgagggctcttcctggtcttctgagggctgcttttgggggttgggggtctgctcccggagcctttggatctctcagaggaactcagagtatcttcagactcagaactgtcaccatctgagaagagggataatcggggagaggtgacggtgctggaccatttcactttcttaggagaggtttcaaaactggagttcagccctctctttgagccttggaaggatgacacatgtggattgacaaaggtctgggaccctacatgctcctctacaggcaaagaatttccacagtaggggcagaatttgaatgccgcttggatacttttgccacagtctggacagaaggagatcatgctttatgaggtcacggtctggcccttggatttactgggttggaaactccatcttgacagcgacctcagcgcaggtggggcgattgcctaggcgacgacagagcctcccttcggccgcacctccatagaaaccacgggatgacttagacgccaagtttcacagcggaggagctgtcgaacttcccacaagttccgcccatctccgccttagccatgcccaacacggagcccaaggtggcttgggaagctcaagaggaggccagtgaaccccgcgacccggagccgctctcattccgaaccccgacagcaggggcctccgcctcccacaaacggtcgtgctgacgtcacggacgccccggccgagctgcggctagggggtcgggggacgtcccctcgttcgcctcgcttcccctcacctctgtacttggggactggggtgggattctgggcttctgcagcctgaccctcggatcctccgcagttaccc

SEQ ID NO: 9260 - RNA, 1830 nt, Homo sapiens
  source 1..1830: mol_type = other RNA
agagctggctgaagggcaggccaccaagatggggaacttcacattcacgggagggaaactggggccctccgggaggctaatcaggactgatgagtatcctgaaaccagtggcaggaatgcacattccagggcttgttctagaagcttatctgtgattaaacagcaggccttgagtcacattacttcatttttttttttctgttgcacactgcaaatggaaagttctggattccacctagggcaccatcgggaggccaatggggtcatatggagacacacgcagatcctgcagcaaagcttctaggttgttcctcagcatggcgtagggcggcttctcctcatacgtgagggccatcaccaccttcaggtacttctgcagggtctctgagggcctgatccagtgaccgcagggtcccacgaagggccccggcttatcaacaaacttctgtttttgcttcatgatgtcctcagtgttgggaaggcaatttgtccatggcagaaacccgtagagccacttcagcatgcagtagcccaggctctggaggtcgctgcggcgggagggcccgcatcccttgtgcaggtccatgctaatgaactcaaggtccccctcgtgagggctcctgctgccttccacgtaggccacgtgtttgccacttgggcaatagcggaaggcgaagccatagcctgccaaagtcacctgactctggtcctctggatccacaaagatattttcagctgtcacatttccatgaacatactcattctcatggaggaactccagggcatccagcagccggcaggccacctgcagcacagacctctctgacagcacatgctttgggctgacatccagggccgactgaaggctcctccccaggctgggtaacaccaagaacctgtatttgtcctggtgaacaccgaaacccatgcaggtagggatggccagcagtggggtcgagtacagcttcttccacttgttgacttgcagaggcttggcggcccgctggaagaagttctgctcattgaacaagcgcccatccttggcatccagtttgagtgagaacttttgcttctgtggtcctgagtcacaggtgagggtggaggtgggtgcagcttcatagagaatgccctggttgtccctggtctggaaggacttcagcttccactgtcgcccactcttgtctgtcagcactgtccctgtgggcaaagcttcaagtgaggtggtcactcggctccgcttcagcgtctgagggctctgcctggtcttctgagggctacagctggtcttctgagggctacccctggtcacctgagggctcttcctggtcttctgagggctgcttttgggggttgggggtctgctcccggagcctttggatctctcagaggaactcagagtatcttcagactcagaactgtcaccatctgagaagagggataatcggggagaggtgacggtgctggaccatttcactttcttaggagaggtttcaaaactggagttcagccctctctttgagccttggaaggatgacacatgtggattgacaaaggtctgggaccctacatgctcctctacaggcaaagaatttccacagtaggggcagaatttgaatgccgcttggatacttttgccacagtctggacagaaggagatcatgctttatgaggtcacggtctggcccttggatttactgggttggaaactccatcttgacagcgacctctgtacttggggactggggtgggattctgggcttctgcagcctgaccctcggatcctccgcagttacccggactcaccttctcagttgcccagcgaaaacttcc

SEQ ID NO: 9261 - RNA, 1751 nt, Homo sapiens
  source 1..1751: mol_type = other RNA
agagctggctgaagggcaggccaccaagatggggaacttcacattcacgggagggaaactggggccctccgggaggctaatcaggactgatgagtatcctgaaaccagtggcaggaatgcacattccagggcttgttctagaagcttatctgtgattaaacagcaggccttgagtcacattacttcatttttttttttctgttgcacactgcaaatggaaagttctggattccacctagggcaccatcgggaggccaatggggtcatatggagacacacgcagatcctgcagcaaagcttctaggttgttcctcagcatggcgtagggcggcttctcctcatacgtgagggccatcaccaccttcaggtacttctgcagggtctctgagggcctgatccagtgaccgcagggtcccacgaagggccccggcttatcaacaaacttctgtttttgcttcatgatgtcctcagtgttgggaaggcaatttgtccatggcagaaacccgtagagccacttcagcatgcagtagcccaggctctggaggtcgctgcggcgggagggcccgcatcccttgtgcaggtccatgctaatgaactcaaggtccccctcgtgagggctcctgctgccttccacgtaggccacgtgtttgccacttgggcaatagcggaaggcgaagccatagcctgccaaagtcacctgactctggtcctctggatccacaaagatattttcagctgtcacatttccatgaacatactcattctcatggaggaactccagggcatccagcagccggcaggccacctgcagcacagacctctctgacagcacatgctttgggctgacatccagggccgactgaaggctcctccccaggctgggtaacaccaagaacctgtatttgtcctggtgaacaccgaaacccatgcaggtagggatggccagcagtggggtcgagtacagcttcttccacttgttgacttgcagaggcttggcggcccgctggaagaagttctgctcattgaacaagcgcccatccttggcatccagtttgagtgagaacttttgcttctgtggtcctgagtcacaggtgagggtggaggtgggtgcagcttcatagagaatgccctggttgtccctggtctggaaggacttcagcttccactgtcgcccactcttgtctgtcagcactgtccctgtgggcaaagcttcaagtgaggtggtcactcggctccgcttcagcgtctgagggctctgcctggtcttctgagggctacagctggtcttctgagggctacccctggtcacctgagggctcttcctggtcttctgagggctgcttttgggggttgggggtctgctcccggagcctttggatctctcagaggaactcagagtatcttcagactcagaactgtcaccatctgagaagagggataatcggggagaggtgacggtgctggaccatttcactttcttaggagaggtttcaaaactggagttcagccctctctttgagccttggaaggatgacacatgtggattgacaaaggtctgggaccctacatgctcctctacaggcaaagaatttccacagtaggggcagaatttgaatgccgcttggatacttttgccacagtctggacagaaggagatcatgctttatgaggtcacggtctggcccttggatttactgggttggaaactccatcttgacagcgaccttctcagttgcccagcgaaaacttcc

SEQ ID NO: 9262 - RNA, 2658 nt, Homo sapiens
  source 1..2658: mol_type = other RNA
agaggctgagaaggtgatgttgaatccttcatatgacatggagaaatcagagatgaagcggacctgggcagtgaagttgccatagagcccagcgctgatgggagctggcagccgagatccagttagctgcctcaggggctgggtgaagctgccgttctcagtgatgaggaggtagtcatggccactttccaggtggaaggtgtggaaagtgaagaacacacccttgccatgagatgtttcgataatccaggtgcagttcaagttgttggggtagaagtcagggaaccctggcgacaagatggtcccactggagccttgaatgaagccaccacagagagcttcacaactgggcagggcccggctccactggaagttgggctcacactccagaggctccccgtcacttaatgtgtagcccgagtcacagctgaaggtcaccagcgcgcccacgtagaagtcattcccatgacgctgtccatttactgggattcctggatccagacagtggtctgactgcagtgttatagtctcatagcggagctggaagccgatgtccgagtgactcttgtcggtagagaagaggaggtagaggtagttgctggtgctgatgaggaactggggaacctgggtcccgtggtaaaccccgatcaagggcgctgagtaagtccgcccatcgcgtacttccagggtgtcatagttgacctcggttttgaatctgtcgaaggtgattttgatggggtagcctggctgggcctcaatcacccaggcacagctcaaggcatccttgtagaagccaggccagcccggagagaggatggtgccgctgggcgaagtcaggtgaccaccacagggagcttcacaccgcagcacagcgctgttccagaccacgctgccctccttcaggacgcaggtgatggtctctgagccctgagtcccaaggaagccttcatcacagaggaaggagatggagctgcccagctggaggctgtccccaaaccgtttgccatttactggaacgccaggatccgggcactcgttgtgtcggaaggtggtaaaagtgatgttgaagcccctcttccctgtggagtggtcagtctggaactcgagacgggccacgtggccactgcttgtgatggaggagggaagctggtttcctgagaaggtgcccaggacgggcgcctcggcggtggccccatccttgatgaccaggaaatcaaactgaggctccacgtcaatgtcgttgaaggccaggtggatgcggctctcaggcctggccaggatgagccagacacagtggaggtggttgccatagtcctctgggtagttgggagacaggacaaccccagacgggctggtgaagttgaagaagcaggagaacacagacgtcttctggctgttgtctttgctgggcatcagcttcacacctcgagacttcaactcaatttgcttcttgacttggtattgggcactgaatccgcgctgccggtggttgccatccgatgtgaagtgcagtcgcagccagttcttgctgctgataacgggggctgggaggctggctccggtgaaccagagggaggagccttctgtcccagtgacttccagaaagtcgtaaccatcctccagctggaagtcaataaacaccagggcgatggtgtcccccagctcagccaggatggtccatgtgcagtcggcattgttatggtactccgaggggaagtgggggctggagatgatgccactctggccccgcagggtcccaccacaggcatcatcagctctgcaggaaggcagggggaagtcccacgtggcgctgttctcagagccagcgtggcaggtgagcacggcgtggccctccaggaagaagccaaggttgcagctgtagcggaccttgtcaccgaggttgaaggttgaaccctgctggatgccattgggcagcctccctgggttcccacatgtgtggctggggagaacttcataggtggcgtggaagccttgggcactgactgcatagtcgctgatgaggcgcagagagagggtggtggctgcactaacaatggtggctggcagctgaaagcctgtgagcctcgtacgcagattctctggctggggtggaccatcaaacaccgacaggacatcaaagtcctcttccagggcaaaggactggaacacaagctggattctgtgctgctcttccgcggtgatggtccacgtgcagttggcgtaattggggtagccatatgggaaccctgggctctcaactgtcccattgggaccgtgcagttggaacgtgcagttctggcccgcggcggccgagacgctgagcaacccacagcccagcaacagcagcagaggcggcggcgttggcggcggcgggcggccccagcggctcccggcgcccggcacaagcgccgaaatcccggtttcgccgcgagccctccccgcggggcagccgcagcgccccagctcccgtccccgcgagcgcggcatggcgcggccggcagcgccgagggagaggctccgctcgccgccgaggagaaaggaggtcaggagagctctggagcttttttctgctcggaaaaaatcccggtacgcgggagccctgagcttctgcggctggaatgaaccaagtgtccgcccggccggggagaggcgcgctgc

SEQ ID NO: 9263 - RNA, 3131 nt, Homo sapiens
  source 1..3131: mol_type = other RNA
agaggctgagaaggtgatgttgaatccttcatatgacatggagaaatcagagatgaagcggacctgggcagtgaagttgccatagagcccagcgctgatgggagctggcagccgagatccagttagctgcctcaggggctgggtgaagctgccgttctcagtgatgaggaggtagtcatggccactttccaggtggaaggtgtggaaagtgaagaacacacccttgccatgagatgtttcgataatccaggtgcagttcaagttgttggggtagaagtcagggaaccctggcgacaagatggtcccactggagccttgaatgaagccaccacagagagcttcacaactgggcagggcccggctccactggaagttgggctcacactccagaggctccccgtcacttaatgtgtagcccgagtcacagctgaaggtcaccagcgcgcccacgtagaagtcattcccatgacgctgtccatttactgggattcctggatccagacagtggtctgactgcagtgttatagtctcatagcggagctggaagccgatgtccgagtgactcttgtcggtagagaagaggaggtagaggtagttgctggtgctgatgaggaactggggaacctgggtcccgtggtaaaccccgatcaagggcgctgagtaagtccgcccatcgcgtacttccagggtgtcatagttgacctcggttttgaatctgtcgaaggtgattttgatggggtagcctggctgggcctcaatcacccaggcacagctcaaggcatccttgtagaagccaggccagcccggagagaggatggtgccgctgggcgaagtcaggtgaccaccacagggagcttcacaccgcagcacagcgctgttccagaccacgctgccctccttcaggacgcaggtgatggtctctgagccctgagtcccaaggaagccttcatcacagaggaaggagatggagctgcccagctggaggctgtccccaaaccgtttgccatttactggaacgccaggatccgggcactcgttgtgtcggaaggtggtaaaagtgatgttgaagcccctcttccctgtggagtggtcagtctggaactcgagacgggccacgtggccactgcttgtgatggaggagggaagctggtttcctgagaaggtgcccaggacgggcgcctcggcggtggccccatccttgatgaccaggaaatcaaactgaggctccacgtcaatgtcgttgaaggccaggtggatgcggctctcaggcctggccaggatgagccagacacagtggaggtggttgccatagtcctctgggtagttgggagacaggacaaccccagacgggctggtgaagttgaagaagcaggagaacacgcagcctggcttcttagccgaccattggttattcttttggcatgtgattgccttctgtcccaccagctcaaaggcgggctggcactcaaacttgagtgtgtcaccgtggtgaaaccgggagccttccctccggccatatgcaggtatgccagggtcaccgcaactgccctgctcgatctcttcataagaagccttgaatcccagggaactgccactgccatcagtctggaagaggagccacatttgatgattggtgctgacaatgagatccgggaccgatgtacctgtcaggatgtagagaactgtcttctggtccccatcctgaccaccatcaccgaccgtcagggtgtcatagcccctctccaaatcaaactcctcaaaggcgagcttgatcaccttggaggggttgagtgctgtgatgatccacacacagtgtgcattgttgtcatactgaatggggaaattgggggaggtgatgatgcccgaggggcctcgaaggtgggcatcacacatgcgggctcggcagactggcctgtggtcgctccaggccgcaaacatgtcgctcactttcatacaggtgatccgcttggacccttgcaggtcatagccctcgttgcaggtgaactggacgctggatcctaacctgaaatccgagcctagtcttttgcccctttcgggtatgccagggtctggacacatattatgtccttgggacacaccaacctgagttaacacagacgtcttctggctgttgtctttgctgggcatcagcttcacacctcgagacttcaactcaatttgcttcttgacttggtattgggcactgaatccgcgctgccggtggttgccatccgatgtgaagtgcagtcgcagccagttcttgctgctgataacgggggctgggaggctggctccggtgaaccagagggaggagccttctgtcccagtgacttccagaaagtcgtaaccatcctccagctggaagtcaataaacaccagggcgatggtgtcccccagctcagccaggatggtccatgtgcagtcggcattgttatggtactccgaggggaagtgggggctggagatgatgccactctggccccgcagggtcccaccacaggcatcatcagctctgcaggaaggcagggggaagtcccacgtggcgctgttctcagagccagcgtggcaggtgagcacggcgtggccctccaggaagaagccaaggttgcagctgtagcggaccttgtcaccgaggttgaaggttgaaccctgctggatgccattgggcagcctccctgggttcccacatgtgtggctggggagaacttcataggtggcgtggaagccttgggcactgactgcatagtcgctgatgaggcgcagagagagggtggtggctgcactaacaatggtggctggcagctgaaagcctgtgagcctcgtacgcagattctctggctggggtggaccatcaaacaccgacaggacatcaaagtcctcttccagggcaaaggactggaacacaagctggattctgtgctgctcttccgcggtgatggtccacgtgcagttggcgtaattggggtagccatatgggaaccctgggctctcaactgtcccattgggaccgtgcagttggaacgtgcagttctggccagctgatcttgggtggtggctttgaacttgccatctagggccgggggcgatgcttatgagcctcattcacaatagcctcctaccccatcccagga

SEQ ID NO: 9264 - RNA, 3222 nt, Homo sapiens
  source 1..3222: mol_type = other RNA
agaggctgagaaggtgatgttgaatccttcatatgacatggagaaatcagagatgaagcggacctgggcagtgaagttgccatagagcccagcgctgatgggagctggcagccgagatccagttagctgcctcaggggctgggtgaagctgccgttctcagtgatgaggaggtagtcatggccactttccaggtggaaggtgtggaaagtgaagaacacacccttgccatgagatgtttcgataatccaggtgcagttcaagttgttggggtagaagtcagggaaccctggcgacaagatggtcccactggagccttgaatgaagccaccacagagagcttcacaactgggcagggcccggctccactggaagttgggctcacactccagaggctccccgtcacttaatgtgtagcccgagtcacagctgaaggtcaccagcgcgcccacgtagaagtcattcccatgacgctgtccatttactgggattcctggatccagacagtggtctgactgcagtgttatagtctcatagcggagctggaagccgatgtccgagtgactcttgtcggtagagaagaggaggtagaggtagttgctggtgctgatgaggaactggggaacctgggtcccgtggtaaaccccgatcaagggcgctgagtaagtccgcccatcgcgtacttccagggtgtcatagttgacctcggttttgaatctgtcgaaggtgattttgatggggtagcctggctgggcctcaatcacccaggcacagctcaaggcatccttgtagaagccaggccagcccggagagaggatggtgccgctgggcgaagtcaggtgaccaccacagggagcttcacaccgcagcacagcgctgttccagaccacgctgccctccttcaggacgcaggtgatggtctctgagccctgagtcccaaggaagccttcatcacagaggaaggagatggagctgcccagctggaggctgtccccaaaccgtttgccatttactggaacgccaggatccgggcactcgttgtgtcggaaggtggtaaaagtgatgttgaagcccctcttccctgtggagtggtcagtctggaactcgagacgggccacgtggccactgcttgtgatggaggagggaagctggtttcctgagaaggtgcccaggacgggcgcctcggcggtggccccatccttgatgaccaggaaatcaaactgaggctccacgtcaatgtcgttgaaggccaggtggatgcggctctcaggcctggccaggatgagccagacacagtggaggtggttgccatagtcctctgggtagttgggagacaggacaaccccagacgggctggtgaagttgaagaagcaggagaacacgcagcctggcttcttagccgaccattggttattcttttggcatgtgattgccttctgtcccaccagctcaaaggcgggctggcactcaaacttgagtgtgtcaccgtggtgaaaccgggagccttccctccggccatatgcaggtatgccagggtcaccgcaactgccctgctcgatctcttcataagaagccttgaatcccagggaactgccactgccatcagtctggaagaggagccacatttgatgattggtgctgacaatgagatccgggaccgatgtacctgtcaggatgtagagaactgtcttctggtccccatcctgaccaccatcaccgaccgtcagggtgtcatagcccctctccaaatcaaactcctcaaaggcgagcttgatcaccttggaggggttgagtgctgtgatgatccacacacagtgtgcattgttgtcatactgaatggggaaattgggggaggtgatgatgcccgaggggcctcgaaggtgggcatcacacatgcgggctcggcagactggcctgtggtcgctccaggccgcaaacatgtcgctcactttcatacaggtgatccgcttggacccttgcaggtcatagccctcgttgcaggtgaactggacgctggatcctaacctgaaatccgagcctagtcttttgcccctttcgggtatgccagggtctggacacatattatgtccttgggacacaccaacctgagttaacacagacgtcttctggctgttgtctttgctgggcatcagcttcacacctcgagacttcaactcaatttgcttcttgacttggtattgggcactgaatccgcgctgccggtggttgccatccgatgtgaagtgcagtcgcagccagttcttgctgctgataacgggggctgggaggctggctccggtgaaccagagggaggagccttctgtcccagtgacttccagaaagtcgtaaccatcctccagctggaagtcaataaacaccagggcgatggtgtcccccagctcagccaggatggtccatgtgcagtcggcattgttatggtactccgaggggaagtgggggctggagatgatgccactctggccccgcagggtcccaccacaggcatcatcagctctgcaggaaggcagggggaagtcccacgtggcgctgttctcagagccagcgtggcaggtgagcacggcgtggccctccaggaagaagccaaggttgcagctgtagcggaccttgtcaccgaggttgaaggttgaaccctgctggatgccattgggcagcctccctgggttcccacatgtgtggctggggagaacttcataggtggcgtggaagccttgggcactgactgcatagtcgctgatgaggcgcagagagagggtggtggctgcactaacaatggtggctggcagctgaaagcctgtgagcctcgtacgcagattctctggctggggtggaccatcaaacaccgacaggacatcaaagtcctcttccagggcaaaggactggaacacaagctggattctgtgctgctcttccgcggtgatggtccacgtgcagttggcgtaattggggtagccatatgggaaccctgggctctcaactgtcccattgggaccgtgcagttggaacgtgcagttctggcccgcggcggccgagacgctgagcaacccacagcccagcaacagcagcagaggcggcggcgttggcggcggcgggcggccccagcggctcccggcgcccggcacaagcgccgaaatcccggtttcgccgcgagccctccccgcggggcagccgcagcgccccagctcccgtccccgcgagcgcggcat

SEQ ID NO: 9265 - RNA, 3355 nt, Homo sapiens
  source 1..3355: mol_type = other RNA
agaggctgagaaggtgatgttgaatccttcatatgacatggagaaatcagagatgaagcggacctgggcagtgaagttgccatagagcccagcgctgatgggagctggcagccgagatccagttagctgcctcaggggctgggtgaagctgccgttctcagtgatgaggaggtagtcatggccactttccaggtggaaggtgtggaaagtgaagaacacacccttgccatgagatgtttcgataatccaggtgcagttcaagttgttggggtagaagtcagggaaccctggcgacaagatggtcccactggagccttgaatgaagccaccacagagagcttcacaactgggcagggcccggctccactggaagttgggctcacactccagaggctccccgtcacttaatgtgtagcccgagtcacagctgaaggtcaccagcgcgcccacgtagaagtcattcccatgacgctgtccatttactgggattcctggatccagacagtggtctgactgcagtgttatagtctcatagcggagctggaagccgatgtccgagtgactcttgtcggtagagaagaggaggtagaggtagttgctggtgctgatgaggaactggggaacctgggtcccgtggtaaaccccgatcaagggcgctgagtaagtccgcccatcgcgtacttccagggtgtcatagttgacctcggttttgaatctgtcgaaggtgattttgatggggtagcctggctgggcctcaatcacccaggcacagctcaaggcatccttgtagaagccaggccagcccggagagaggatggtgccgctgggcgaagtcaggtgaccaccacagggagcttcacaccgcagcacagcgctgttccagaccacgctgccctccttcaggacgcaggtgatggtctctgagccctgagtcccaaggaagccttcatcacagaggaaggagatggagctgcccagctggaggctgtccccaaaccgtttgccatttactggaacgccaggatccgggcactcgttgtgtcggaaggtggtaaaagtgatgttgaagcccctcttccctgtggagtggtcagtctggaactcgagacgggccacgtggccactgcttgtgatggaggagggaagctggtttcctgagaaggtgcccaggacgggcgcctcggcggtggccccatccttgatgaccaggaaatcaaactgaggctccacgtcaatgtcgttgaaggccaggtggatgcggctctcaggcctggccaggatgagccagacacagtggaggtggttgccatagtcctctgggtagttgggagacaggacaaccccagacgggctggtgaagttgaagaagcaggagaacacgcagcctggcttcttagccgaccattggttattcttttggcatgtgattgccttctgtcccaccagctcaaaggcgggctggcactcaaacttgagtgtgtcaccgtggtgaaaccgggagccttccctccggccatatgcaggtatgccagggtcaccgcaactgccctgctcgatctcttcataagaagccttgaatcccagggaactgccactgccatcagtctggaagaggagccacatttgatgattggtgctgacaatgagatccgggaccgatgtacctgtcaggatgtagagaactgtcttctggtccccatcctgaccaccatcaccgaccgtcagggtgtcatagcccctctccaaatcaaactcctcaaaggcgagcttgatcaccttggaggggttgagtgctgtgatgatccacacacagtgtgcattgttgtcatactgaatggggaaattgggggaggtgatgatgcccgaggggcctcgaaggtgggcatcacacatgcgggctcggcagactggcctgtggtcgctccaggccgcaaacatgtcgctcactttcatacaggtgatccgcttggacccttgcaggtcatagccctcgttgcaggtgaactggacgctggatcctaacctgaaatccgagcctagtcttttgcccctttcgggtatgccagggtctggacacatattatgtccttgggacacaccaacctgagttaacacagacgtcttctggctgttgtctttgctgggcatcagcttcacacctcgagacttcaactcaatttgcttcttgacttggtattgggcactgaatccgcgctgccggtggttgccatccgatgtgaagtgcagtcgcagccagttcttgctgctgataacgggggctgggaggctggctccggtgaaccagagggaggagccttctgtcccagtgacttccagaaagtcgtaaccatcctccagctggaagtcaataaacaccagggcgatggtgtcccccagctcagccaggatggtccatgtgcagtcggcattgttatggtactccgaggggaagtgggggctggagatgatgccactctggccccgcagggtcccaccacaggcatcatcagctctgcaggaaggcagggggaagtcccacgtggcgctgttctcagagccagcgtggcaggtgagcacggcgtggccctccaggaagaagccaaggttgcagctgtagcggaccttgtcaccgaggttgaaggttgaaccctgctggatgccattgggcagcctccctgggttcccacatgtgtggctggggagaacttcataggtggcgtggaagccttgggcactgactgcatagtcgctgatgaggcgcagagagagggtggtggctgcactaacaatggtggctggcagctgaaagcctgtgagcctcgtacgcagattctctggctggggtggaccatcaaacaccgacaggacatcaaagtcctcttccagggcaaaggactggaacacaagctggattctgtgctgctcttccgcggtgatggtccacgtgcagttggcgtaattggggtagccatatgggaaccctgggctctcaactgtcccattgggaccgtgcagttggaacgtgcagttctggcccgcggcggccgagacgctgagcaacccacagcccagcaacagcagcagaggcggcggcgttggcggcggcgggcggccccagcggctcccggcgcccggcacaagcgccgaaatcccggtttcgccgcgagccctccccgcggggcagccgcagcgccccagctcccgtccccgcgagcgcggcatggcgcggccggcagcgccgagggagaggctccgctcgccgccgaggagaaaggaggtcaggagagctctggagcttttttctgctcggaaaaaatcccggtacgcgggagccctgagcttctgcggctggaat

SEQ ID NO: 9266 - RNA, 3393 nt, Homo sapiens
  source 1..3393: mol_type = other RNA
agaggctgagaaggtgatgttgaatccttcatatgacatggagaaatcagagatgaagcggacctgggcagtgaagttgccatagagcccagcgctgatgggagctggcagccgagatccagttagctgcctcaggggctgggtgaagctgccgttctcagtgatgaggaggtagtcatggccactttccaggtggaaggtgtggaaagtgaagaacacacccttgccatgagatgtttcgataatccaggtgcagttcaagttgttggggtagaagtcagggaaccctggcgacaagatggtcccactggagccttgaatgaagccaccacagagagcttcacaactgggcagggcccggctccactggaagttgggctcacactccagaggctccccgtcacttaatgtgtagcccgagtcacagctgaaggtcaccagcgcgcccacgtagaagtcattcccatgacgctgtccatttactgggattcctggatccagacagtggtctgactgcagtgttatagtctcatagcggagctggaagccgatgtccgagtgactcttgtcggtagagaagaggaggtagaggtagttgctggtgctgatgaggaactggggaacctgggtcccgtggtaaaccccgatcaagggcgctgagtaagtccgcccatcgcgtacttccagggtgtcatagttgacctcggttttgaatctgtcgaaggtgattttgatggggtagcctggctgggcctcaatcacccaggcacagctcaaggcatccttgtagaagccaggccagcccggagagaggatggtgccgctgggcgaagtcaggtgaccaccacagggagcttcacaccgcagcacagcgctgttccagaccacgctgccctccttcaggacgcaggtgatggtctctgagccctgagtcccaaggaagccttcatcacagaggaaggagatggagctgcccagctggaggctgtccccaaaccgtttgccatttactggaacgccaggatccgggcactcgttgtgtcggaaggtggtaaaagtgatgttgaagcccctcttccctgtggagtggtcagtctggaactcgagacgggccacgtggccactgcttgtgatggaggagggaagctggtttcctgagaaggtgcccaggacgggcgcctcggcggtggccccatccttgatgaccaggaaatcaaactgaggctccacgtcaatgtcgttgaaggccaggtggatgcggctctcaggcctggccaggatgagccagacacagtggaggtggttgccatagtcctctgggtagttgggagacaggacaaccccagacgggctggtgaagttgaagaagcaggagaacacgcagcctggcttcttagccgaccattggttattcttttggcatgtgattgccttctgtcccaccagctcaaaggcgggctggcactcaaacttgagtgtgtcaccgtggtgaaaccgggagccttccctccggccatatgcaggtatgccagggtcaccgcaactgccctgctcgatctcttcataagaagccttgaatcccagggaactgccactgccatcagtctggaagaggagccacatttgatgattggtgctgacaatgagatccgggaccgatgtacctgtcaggatgtagagaactgtcttctggtccccatcctgaccaccatcaccgaccgtcagggtgtcatagcccctctccaaatcaaactcctcaaaggcgagcttgatcaccttggaggggttgagtgctgtgatgatccacacacagtgtgcattgttgtcatactgaatggggaaattgggggaggtgatgatgcccgaggggcctcgaaggtgggcatcacacatgcgggctcggcagactggcctgtggtcgctccaggccgcaaacatgtcgctcactttcatacaggtgatccgcttggacccttgcaggtcatagccctcgttgcaggtgaactggacgctggatcctaacctgaaatccgagcctagtcttttgcccctttcgggtatgccagggtctggacacatattatgtccttgggacacaccaacctgagttaacacagacgtcttctggctgttgtctttgctgggcatcagcttcacacctcgagacttcaactcaatttgcttcttgacttggtattgggcactgaatccgcgctgccggtggttgccatccgatgtgaagtgcagtcgcagccagttcttgctgctgataacgggggctgggaggctggctccggtgaaccagagggaggagccttctgtcccagtgacttccagaaagtcgtaaccatcctccagctggaagtcaataaacaccagggcgatggtgtcccccagctcagccaggatggtccatgtgcagtcggcattgttatggtactccgaggggaagtgggggctggagatgatgccactctggccccgcagggtcccaccacaggcatcatcagctctgcaggaaggcagggggaagtcccacgtggcgctgttctcagagccagcgtggcaggtgagcacggcgtggccctccaggaagaagccaaggttgcagctgtagcggaccttgtcaccgaggttgaaggttgaaccctgctggatgccattgggcagcctccctgggttcccacatgtgtggctggggagaacttcataggtggcgtggaagccttgggcactgactgcatagtcgctgatgaggcgcagagagagggtggtggctgcactaacaatggtggctggcagctgaaagcctgtgagcctcgtacgcagattctctggctggggtggaccatcaaacaccgacaggacatcaaagtcctcttccagggcaaaggactggaacacaagctggattctgtgctgctcttccgcggtgatggtccacgtgcagttggcgtaattggggtagccatatgggaaccctgggctctcaactgtcccattgggaccgtgcagttggaacgtgcagttctggcccgcggcggccgagacgctgagcaacccacagcccagcaacagcagcagaggcggcggcgttggcggcggcgggcggccccagcggctcccggcgcccggcacaagcgccgaaatcccggtttcgccgcgagccctccccgcggggcagccgcagcgccccagctcccgtccccgcgagcgcggcatggcgcggccggcagcgccgagggagaggctccgctcgccgccgaggagaaaggaggtcaggagagctctggagcttttttctgctcggaaaaaatcccggtacgcgggagccctgagcttctgcggctggaatgaaccaagtgtccgcccggccggggagaggcgcgctgc

SEQ ID NO: 9267 - RNA, 2383 nt, Homo sapiens
  source 1..2383: mol_type = other RNA
agaggctgagaaggtgatgttggctgtcttgtcaaaaggtgcgttcacactctcctcctgctccccaaactcctcatcattgaagccgaagtggtcaatgaaggcagaggtcatgcgctgcatctggaagtccatgaaggcctgctgcagcacagcctcctcagggaagttgaactccttgagccggtcgtcctcatcgtcactggaggagtgtaggtggtgggtgttcaccaggtccaccatgttcttcttgttggtctccgccaggggccccgatacgaaggcttcccactgctcctgctgctcgctgggcagctccttcagcagctgccgcagctgctctgcattgggccccttctccgtgttctgcaccagggcaccggccactcttgtcaggtgacccatgtagcctttccgagggcctcccgcacactgtacacggtcgttctcctcccaggacgtcaggatccgctccaccaggcggcactgctgcagcagatgtttcacaacagggttttggatgggcgtctcagggctgctgtcaggaggtggccccaagctcagcatggtgctcacgcatccctctacttgggcatgcaagaagttgttgaagacataatggaagaagaggtccagcatggtgttgggcacgtccagtgccaggagctcgtgcgtcagggctgcatcattggcgctcagggcactggccaggagcttgaccacgtgcagccgcgtgttgcccagaggcggagccagcatgccccatgtcatctgtagcggctccagcttgggaggctccagcaggagctggtggaagcagctgagccgcgggcgtagggcgtgcaaggcgcccacactggacacagtgctttccagggccccctgggccaggagctccagctgcccatccacactgctgaagaagctgttcacggtcacggactcggacctcggcctcctgggctccagcagggtcagcagcacctggatcccactgacgatgacagactggctctgctccccctcgaacatgttgcttaagagctgctcaatcgtctcctgcttctccagggtggccagcagttggtcaggctctgggctgtcctggacttggatcatctgctcccggctcaggcggatgatgtcacacagggactgggatgcgttggaatgttgattctcatccttcgacgggtggatctgctcaatcagccgctggacgatcttctcctcgttgagccaattgacaacatcctgcctcagctgaggccgctccacacaggtgagcaggcgcagcaggaggtccatgatggccgaggtgccaatgtgctgcagcagcaggtccacgaagtcatccttcttccgaagaaaggacacgagctggtctgtcttgcggttgatgaggatgcccatgaccttgctgaagaagctggccagcagtgggttgaggctgccggtgctctgcaggaagccgtagagccggttcagaagggactcatcagcacccagggcatcattgatctggggcacatctgaggtcagaatctcgcaggccacactggggtacttgtagcgcagccgctcctcaccgctatctggcggctcctgggtgacccaggccaccattgcttgcaggtggggtggctgcagcaggaagtccagcagcttgcggttgacgaccttgcactcctgcagcacgtcttcctcgtccagcagctcgggcaggctcaggtcctcccgctccagcagcgtgtccaggtgcgagcttgtgtgcaggtcaaacttccaaaacatggcgccctgcgagggggggcggcggctcctcgcactcggggctcatcggggcgcccccccccgccccgccgccggcggctccggcccctgctgcggggcccggtgagtgggggcgggggcggcgtcggggactcgcgcaggcgccggggctcgcggggtccgcgcaggcgcccgcgggtcgtggggtcctcgcgcgccgggtcctgcagagttgagggggtcagcgccgggtggagttgccgacgggcggggggcgtcactagtccgcgtaggcacctccggggtccgcaggcgaggtgggcgtgcgggccgaggcgggttggcgagccgggtcgcgaggcccacgcaggcgcctcagccgggaagacgggggaagttgccccggtttccacagtccaaccgagcgccccacgggaggggaaggcgacctcctccgcggtccaaacgggccgcagagccgagcagcgaccgacggaagccgaggcctacttccttaaccaccccttccccaaagccgctcaatctccgggctctgcggccggcctcagggcctccgacgcccggctccctccgccactatcccacaatc

SEQ ID NO: 9268 - RNA, 538 nt, Homo sapiens
  source 1..538: mol_type = other RNA
agagtcggcgacgccgccagcaggagccagggcagcgcgcagagcagcgcgagccgcaggcagccgcgcatggtgggcaccgcgcccgggctcgaaagcggagccaccctggggagggggcgagcgcagagagggtccttccaaagcccggtgcagggccaggcgtccgcttcagagccgagcgggtgatgcctggcgaacccagccggccagggctggcagcgtgctgacgaagggccgatcaaatactgatgctgccgcctggggtctccactggaggtcacgggtggagagtagggcggactggagaagtggagatgtggggctgctgattttcctccggcttctaagtcccccgtttctcatcgccgagaatccccccacttacccagccagaatttagaccgatctcttctccctcaacctcaataacagcaataataaaaaggcattggagtcattaaaaagaaatacccgctagtctcgaaaagtcaacctgacgccacatcgaggaggaaattcggtctgtttcaaatac

SEQ ID NO: 9269 - RNA, 580 nt, Homo sapiens
  source 1..580: mol_type = other RNA
agagtcggcgacgccgccagcaggagccagggcagcgcgcagagcagcgcgagccgcaggcagccgcgcatggtgggcaccgcgcccgggctcgaaagcggagccaccctggggagggggcgagcgcagagagggtccttccaaagcccggtgcagggccaggcgtccgcttcagagccgagcgggtgatgcctggcgaacccagccggccagggctggcagcgtgctgacgaagggccgatcaaatactgatgctgccgcctggggtctccactggaggtcacgggtggagagtagggcggactggagaagtggagatgtggggctgctgattttcctccggcttctaagtcccccgtttctcatcgccgagaatccccccacttacccagccagaatttagaccgatctcttctccctcaacctcaataacagcaataataaaaaggcattggagtcattaaaaagaaatacccgctagtctcgaaaagtcaacctgacgccacatcgaggaggaaattcggtctgtttcaaatacgtgtgcaccctggctgcaggagaagaaatagaaagcaaaaga

SEQ ID NO: 9270 - RNA, 797 nt, Homo sapiens
  source 1..797: mol_type = other RNA
agagtcggcgacgccgccagcaggagccagggcagcgcgcagagcagcgcgagccgcaggcagccgcgcatggtgggcaccgcgcccgggctcgaaagcggagccaccctggggagggggcgagcgcagagagggtccttccaaagcccggtgcagggccaggcgtccgcttcagagccgagcgggtgatgcctggcgaacccagccggccagggctggcagcgtgctgacgaagggccgatcaaatactgatgctgccgcctggggtctccactggaggtcacgggtggagagtagggcggactggagaagtggagatgtggggctgctgattttcctccggcttctaagtcccccgtttctcatcgccgagaatccccccacttacccagccagaatttagaccgatctcttctccctcaacctcaataacagcaataataaaaaggcattggagtcattaaaaagaaatacccgctagtctcgaaaagtcaacctgacgccacatcgaggaggaaattcggtctgtttcaaatacgtgtgcaccctggctgcaggagaagaaatagaaagcaaaagagcccgtcccccaagagggtgcgcgagttcgctttcccaggctgctacctgcagagaactcttgcctgtctgaacgataattactctctattctcccctctctaatagaacctctcctcagacacctgttttatttctttattacctcctactctccatggagagtctcacgtcatcacgttctctccctcaccatatgtgtatgtatgtaaatatgt

SEQ ID NO: 9271 - RNA, 81 nt, Homo sapiens
  source 1..81: mol_type = other RNA
agatgtccagccacaattctcggttggccgcagactcgtacaagaattgcgtttggacaatcagtggcgaagcccctgagt

SEQ ID NO: 9272 - RNA, 63 nt, Homo sapiens
  source 1..63: mol_type = other RNA
agattgtttcttttgccgtgcaaaaacttaaacttgcacggcaaaagaaacaatctgcaggaa

SEQ ID NO: 9273 - RNA, 114 nt, Homo sapiens
  source 1..114: mol_type = other RNA
agattgtttcttttgccgtgcagaagctctttactttaattaggtcccatttgtcaatttttggttttgttgcaattgcttttggcatcttcatcatggaatctttgccaggaa

SEQ ID NO: 9274 - RNA, 406 nt, Homo sapiens
  source 1..406: mol_type = other RNA
agcaaaataagcaaatggaaaaagatagggtgtgctagggagatcccactctatcccaggcctttgtttcttccctagattactcagccctgtgtgtttatcctaaaggggctctgcagcactggaaatttgtttggcagatgatgtccttttttctccccagcattcactgctctaggcagagacccagggtcacagcaactccccagggccttcacatgtccccagtgtccatgggaactctcctcccagcctttcacacacaccctcctttgctgcctctccaggttccagcagtggcctgaattctcaggagatggatggtatattcccttactggtctaggccagaaaaagggggatgaaaatgtctggataagacagggcaggaaacaggatcaactcca

SEQ ID NO: 9275 - RNA, 410 nt, Homo sapiens
  source 1..410: mol_type = other RNA
agcaaaataagcaaatggaaaaagatagggtgtgctagggagatcccactctatcccaggcctttgtttcttccctagattactcagccctgtgtgtttatcctaaaggggctctgcagcactggaaatttgtttggcagatgatgtccttttttctccccagcattcactgctctaggcagagacccagggtcacagcaactccccagggccttcacatgtccccagtgtccatgggaactctcctcccagcctttcacacacaccctcctttgctgcctctccaggttccagcagtggcctgaattctcaggagatggatggtatattcccttactggtctaggccagaaaaagggggatgaaaatgtctggataagacagggcaggaaacaggatcaactccaagtc

SEQ ID NO: 9276 - RNA, 4308 nt, Homo sapiens
  source 1..4308: mol_type = other RNA
agcagaggcagagaggctcaggagattgtccagggacaaggagacctggccggacctctgcagggaggtgaggcccctgcccccatcttgtcccatcacattctggatgtttggcatccccaggctcctgggaggggagaagtgctgataaaaaggccaaaaatcacacagaaagaagacagaaaactccacgcacttcctacataggtgctaccgtattcctacgagcacggggcctgtgttgaagactccctctggaagttacagaaggaagccaccaagagttcagcctcacagcctctttctcagatgcagtcaccactttaccaaacttggcacatccaaccactcctttcataattttacacctgtttgtggcctggctgacagatattttgtcattgatctttctaatttcagggattctaaatgtgttttgagaatctgctcagcactcagggattctgtctttaaaaatatgattaaaccaccagatagtgtgatttcagaaagtgtgcgtggctaccaaaaacttctaaacacaagttatatgagtgactcctgtcttctgtggctgagcttgggtactgattgtctttctccatgccttgcatcccctgttagaggagggcctgctgtccatggctgtccatgcactttaaaatgtctcaggtttagctgaagaccagatgggtccaagtttatttatatctgctggcataagaatgatggctaaattacctctttaagttgtttttttgtttgtttgttttgacagagtctcgctgtgatgcccaagctggagtgcagtggcatgatcttggctcactgcgacctccgtttcctgggttcaagcgattctcctgcctcagcctcccgagtagctgggactacagacacatgccaccatgcccggctaatttttgtatttttagtagagatggggttttaccatattggccaggctagtctcaaactccttacctcaagtgatccacccgcctcggcctcctaaagtgctgagatgtctctttaactttcaagaggtacagcaaaactgaaatcaatgggtgatgacttcttaaagatcaaacatgaagatgaggattagttaagaccagaaaatcattctccgatcttgtatcttcaactcaaattcacactccaaaaggcctgtttgtggtgaggctcagggtctttggcttgttctgaattaatactttctttggaaactctttagatggctttgatccctgtgctgccccccattgcagacacagaaagcgacaggggattctggcggcaccctctctgtggaggagaggaaggtgtggaccacgttcagaggaaggcagcctgaagctgtcctcagtgagatgctgggggatgggcctcttgcccctgctgtgcagcctccatgcagggctttatttaccagtcaccaggtcttcaagacagtctgcaggagagaggatttcagggggaaagtaagccaagccaattcattctcatggtccccttttatcacaaacatgtaagtcttccatctcataacagagacagcaaaagcagtatccaggccttttttttttttctttctttctttccttaactggctacatgcttagaaactgcactggtcaaacttgattttctttttaaagcctcaaaacatttttattgtcaggaaagcttttcagtggccagggatcagtctcatggccgtagaagcagccaaattcctctgcctttgccttcccttcaggagtcacatgctaaggcatccttgggcatttggaaaaggccgcttggggtgagagtgctctaggccactctgcaatgtccctgggcccgatgagtaacaaatgcaccccgggacccagagaagtggaaagacatgaaagggatttggaaacagatcgtaaaaataacctgtatgaaaatcacacagacaagaaaacaaacaaatccagctagccccttggatcctgccatccgtcttttctcccgggactgcctttgctttgtggagggtgagtcctgggacaggctttgggtgacaagttgtgggcatgttccatccaagcctggctctcccgactggcagagggaggtggctgacaatcaattcctctggatacattttcctgtgattgctcctgtgatcaaaggcagccaccgacaggtgcgggagcggttagttcaccacgtcatagtagtaattgcgcagccgcagttccactgctgcgaatccgggcctgttttccacatcgtatgtccagcacagattcatgagatcgtacatctctcttggacaccctgcagggcaccccatccgctctcctttctctaacatagcggtgacttcacttcctttcatccctcgatatggcttctgcccataggagaatgcttcccacatcaacactccaaagctccagacatcgcttttgctggagaacttgtagtagttgatgcattccggagcgtaccacttgacaggccactttccatgggtctgggccttgtagtagttttcatcagcacgcagtgctttggaaagtccgaaatcactgatcttggcgtaatgttgggtaactagcaacacatttcttgcagccagatctctgtgcacaaaattgctctcctccaagtacttcatgcccatggaaacctgatgaaccagttctatgatgttcttatccttgacatgtctgttctgctgcaaatacttattgaggggaccaagttctgccatctccataaccagcatccaggactcggcctcgcatatcccgatcatccgcacgatgtacgggttgtccagctgctgcatgacatttgcttctgctaataactcatctttaagagcggggtcattggcctcgtttttcagtattttcacagccacggttttcacaacttttttcatttggtagtagccctttttcacagttccaaaattaccagagcccagttctttgtcttccagcgtcagcagctttcggtccaggtaaacctccttgggcctgatctcctcggggtccgcgtaggggctctcgtacacctctgtgtccatgggtagggcttctctctgggggcctttgtctgcagcccagggtgcaagttctggctcatacggattgaatgacacagtactctcttgccggttcccttgggcaggggaggacacttagttggacagcaagcaggggttgctttagcacctttctgtggccaggctttgggaaggagtatgatttgattcttgagattattccacccgctgaccaagtcgcaggatgggaacctggaagttgtggacggcctccaaaattaacatttccctgtgtgccgattttttgacatgggacagtaagaactcttaacaaaccatctgctttataagaataatgctcgactagctgccagagcgtgtcgaacttctttccctcggggatggagagcttccctgtcttgtctttgtcgatgcgatagtgcagcaccttcccttcgtgcagcaggcacagggcgtaggagccgttgttgtctctggctcggatcaggaactttccatttgtctttgatcctatcaggacaatttgctcagattcttcccgagagatttttccatggaaccaaggcattttttcatgggctgtggtagcgatcagcttctccagctgaggcttctgactgatgatggcctgctccagagcctgaccctgcaggttccatgtctgcttcacatattccctgatgaggttttccttcaaatcctcaaagggcccagtcttgggctgcaccccttggggccggttgaagggcttcttgaggaggcagaccaggccatcagactcctgggagtggtagtggcagaggtcggcggggctggcatgggtcctgccaccggcgatggcgtaggtgccattcagctcccgctcgatggtgtagtggtgtgccttcctcccgtgggccacggacagggcgaagccacccaggtagttgcggctctggcgcagcaaataaagcccatcactcatgcccccctggaccaggtaatcttctgcctcctcccgggtgatgttgccgaaaaagaagggcaggtggttggcgctgtcagccatgccgctgctggccatgcttcaggggccggagggcacacacctgcgcaggtgtccacctgcgccaggtgaggcgagggcgggcgcagcgcggggccacccgctcctcctcgctctccagccgccgccggggtggcctcagccgccgggcccgcggctcttcctcattttgggcaacttcctt

SEQ ID NO: 9277 - RNA, 4483 nt, Homo sapiens
  source 1..4483: mol_type = other RNA
agcagaggcagagaggctcaggagattgtccagggacaaggagacctggccggacctctgcagggaggtgaggcccctgcccccatcttgtcccatcacattctggatgtttggcatccccaggctcctgggaggggagaagtgctgataaaaaggccaaaaatcacacagaaagaagacagaaaactccacgcacttcctacataggtgctaccgtattcctacgagcacggggcctgtgttgaagactccctctggaagttacagaaggaagccaccaagagttcagcctcacagcctctttctcagatgcagtcaccactttaccaaacttggcacatccaaccactcctttcataattttacacctgtttgtggcctggctgacagatattttgtcattgatctttctaatttcagggattctaaatgtgttttgagaatctgctcagcactcagggattctgtctttaaaaatatgattaaaccaccagatagtgtgatttcagaaagtgtgcgtggctaccaaaaacttctaaacacaagttatatgagtgactcctgtcttctgtggctgagcttgggtactgattgtctttctccatgccttgcatcccctgttagaggagggcctgctgtccatggctgtccatgcactttaaaatgtctcaggtttagctgaagaccagatgggtccaagtttatttatatctgctggcataagaatgatggctaaattacctctttaagttgtttttttgtttgtttgttttgacagagtctcgctgtgatgcccaagctggagtgcagtggcatgatcttggctcactgcgacctccgtttcctgggttcaagcgattctcctgcctcagcctcccgagtagctgggactacagacacatgccaccatgcccggctaatttttgtatttttagtagagatggggttttaccatattggccaggctagtctcaaactccttacctcaagtgatccacccgcctcggcctcctaaagtgctgagatgtctctttaactttcaagaggtacagcaaaactgaaatcaatgggtgatgacttcttaaagatcaaacatgaagatgaggattagttaagaccagaaaatcattctccgatcttgtatcttcaactcaaattcacactccaaaaggcctgtttgtggtgaggctcagggtctttggcttgttctgaattaatactttctttggaaactctttagatggctttgatccctgtgctgccccccattgcagacacagaaagcgacaggggattctggcggcaccctctctgtggaggagaggaaggtgtggaccacgttcagaggaaggcagcctgaagctgtcctcagtgagatgctgggggatgggcctcttgcccctgctgtgcagcctccatgcagggctttatttaccagtcaccaggtcttcaagacagtctgcaggagagaggatttcagggggaaagtaagccaagccaattcattctcatggtccccttttatcacaaacatgtaagtcttccatctcataacagagacagcaaaagcagtatccaggccttttttttttttctttctttctttccttaactggctacatgcttagaaactgcactggtcaaacttgattttctttttaaagcctcaaaacatttttattgtcaggaaagcttttcagtggccagggatcagtctcatggccgtagaagcagccaaattcctctgcctttgccttcccttcaggagtcacatgctaaggcatccttgggcatttggaaaaggccgcttggggtgagagtgctctaggccactctgcaatgtccctgggcccgatgagtaacaaatgcaccccgggacccagagaagtggaaagacatgaaagggatttggaaacagatcgtaaaaataacctgtatgaaaatcacacagacaagaaaacaaacaaatccagctagccccttggatcctgccatccgtcttttctcccgggactgcctttgctttgtggagggtgagtcctgggacaggctttgggtgacaagttgtgggcatgttccatccaagcctggctctcccgactggcagagggaggtggctgacaatcaattcctctggatacattttcctgtgattgctcctgtgatcaaaggcagccaccgacaggtgcgggagcggttagttcaccacgtcatagtagtaattgcgcagccgcagttccactgctgcgaatccgggcctgttttccacatcgtatgtccagcacagattcatgagatcgtacatctctcttggacaccctgcagggcaccccatccgctctcctttctctaacatagcggtgacttcacttcctttcatccctcgatatggcttctgcccataggagaatgcttcccacatcaacactccaaagctccagacatcgcttttgctggagaacttgtagtagttgatgcattccggagcgtaccacttgacaggccactttccatgggtctgggccttgtagtagttttcatcagcacgcagtgctttggaaagtccgaaatcactgatcttggcgtaatgttgggtaactagcaacacatttcttgcagccagatctctgtgcacaaaattgctctcctccaagtacttcatgcccatggaaacctgatgaaccagttctatgatgttcttatccttgacatgtctgttctgctgcaaatacttattgaggggaccaagttctgccatctccataaccagcatccaggactcggcctcgcatatcccgatcatccgcacgatgtacgggttgtccagctgctgcatgacatttgcttctgctaataactcatctttaagagcggggtcattggcctcgtttttcagtattttcacagccacggttttcacaacttttttcatttggtagtagccctttttcacagttccaaaattaccagagcccagttctttgtcttccagcgtcagcagctttcggtccaggtaaacctccttgggcctgatctcctcggggtccgcgtaggggctctcgtacacctctgtgtccatgggtagggcttctctctgggggcctttgtctgcagcccagggtgcaagttctggctcatacggattgaatgacacagtactctcttgccggttcccttgggcaggggaggacgcaggatgggaacctggaagttgtggacggcctccaaaattaacatttccctgtgtgccgattttttgacatgggacagtaagaactcttaacaaaccatctgctttataagaataatgctcgactagctgccagagcgtgtcgaacttctttccctcggggatggagagcttccctgtcttgtctttgtcgatgcgatagtgcagcaccttcccttcgtgcagcaggcacagggcgtaggagccgttgttgtctctggctcggatcaggaactttccatttgtctttgatcctatcaggacaatttgctcagattcttcccgagagatttttccatggaaccaaggcattttttcatgggctgtggtagcgatcagcttctccagctgaggcttctgactgatgatggcctgctccagagcctgaccctgcaggttccatgtctgcttcacatattccctgatgaggttttccttcaaatcctcaaagggcccagtcttgggctgcaccccttggggccggttgaagggcttcttgaggaggcagaccaggccatcagactcctgggagtggtagtggcagaggtcggcggggctggcatgggtcctgccaccggcgatggcgtaggtgccattcagctcccgctcgatggtgtagtggtgtgccttcctcccgtgggccacggacagggcgaagccacccaggtagttgcggctctggcgcagcaaataaagcccatcactcatgcccccctggaccaggtaatcttctgcctcctcccgggtgatgttgccgaaaaagaagggcaggtggttggcgctgtcagccatgccgctgctggccatgcttcaggggccggagggcacacacctgcgcaggtgtccacctcggccgatgaaggtagaacaagaaagggcatgaaagcagcgcgtcgttccccgtaacctcctctccttaccagaaagtcccggccgggtaggggacgcggccacacctacctgcgccaggtgaggcgagggcgggcgcagcgcggggccacccgctcctcctcgctctccagccgccgccggggtggcctcagccgccgggcccgcggctcttcctcattttgggcaacttccttaacgcgcccgggcaggcggcccgcacttcctcccagtgtcgcgccccgccgccctggcccgccctgctgaccgcgcccatgagcccggagctgggcgggaatcggctgaagcgccgggcgaggcccgcggaatcggcccaggcggcggcaggtgtagaggagcccgggt

SEQ ID NO: 9278 - RNA, 4152 nt, Homo sapiens
  source 1..4152: mol_type = other RNA
agcagaggcagagaggctcaggagattgtccagggacaaggagacctggccggacctctgcagggaggtgaggcccctgcccccatcttgtcccatcacattctggatgtttggcatccccaggctcctgggaggggagaagtgctgataaaaaggccaaaaatcacacagaaagaagacagaaaactccacgcacttcctacataggtgctaccgtattcctacgagcacggggcctgtgttgaagactccctctggaagttacagaaggaagccaccaagagttcagcctcacagcctctttctcagatgcagtcaccactttaccaaacttggcacatccaaccactcctttcataattttacacctgtttgtggcctggctgacagatattttgtcattgatctttctaatttcagggattctaaatgtgttttgagaatctgctcagcactcagggattctgtctttaaaaatatgattaaaccaccagatagtgtgatttcagaaagtgtgcgtggctaccaaaaacttctaaacacaagttatatgagtgactcctgtcttctgtggctgagcttgggtactgattgtctttctccatgccttgcatcccctgttagaggagggcctgctgtccatggctgtccatgcactttaaaatgtctcaggtttagctgaagaccagatgggtccaagtttatttatatctgctggcataagaatgatggctaaattacctctttaagttgtttttttgtttgtttgttttgacagagtctcgctgtgatgcccaagctggagtgcagtggcatgatcttggctcactgcgacctccgtttcctgggttcaagcgattctcctgcctcagcctcccgagtagctgggactacagacacatgccaccatgcccggctaatttttgtatttttagtagagatggggttttaccatattggccaggctagtctcaaactccttacctcaagtgatccacccgcctcggcctcctaaagtgctgagatgtctctttaactttcaagaggtacagcaaaactgaaatcaatgggtgatgacttcttaaagatcaaacatgaagatgaggattagttaagaccagaaaatcattctccgatcttgtatcttcaactcaaattcacactccaaaaggcctgtttgtggtgaggctcagggtctttggcttgttctgaattaatactttctttggaaactctttagatggctttgatccctgtgctgccccccattgcagacacagaaagcgacaggggattctggcggcaccctctctgtggaggagaggaaggtgtggaccacgttcagaggaaggcagcctgaagctgtcctcagtgagatgctgggggatgggcctcttgcccctgctgtgcagcctccatgcagggctttatttaccagtcaccaggtcttcaagacagtctgcaggagagaggatttcagggggaaagtaagccaagccaattcattctcatggtccccttttatcacaaacatgtaagtcttccatctcataacagagacagcaaaagcagtatccaggccttttttttttttctttctttctttccttaactggctacatgcttagaaactgcactggtcaaacttgattttctttttaaagcctcaaaacatttttattgtcaggaaagcttttcagtggccagggatcagtctcatggccgtagaagcagccaaattcctctgcctttgccttcccttcaggagtcacatgctaaggcatccttgggcatttggaaaaggccgcttggggtgagagtgctctaggccactctgcaatgtccctgggcccgatgagtaacaaatgcaccccgggacccagagaagtggaaagacatgaaagggatttggaaacagatcgtaaaaataacctgtatgaaaatcacacagacaagaaaacaaacaaatccagctagccccttggatcctgccatccgtcttttctcccgggactgcctttgctttgtggagggtgagtcctgggacaggctttgggtgacaagttgtgggcatgttccatccaagcctggctctcccgactggcagagggaggtggctgacaatcaattcctctggatacattttcctgtgattgctcctgtgatcaaaggcagccaccgacaggtgcgggagcggttagttcaccacgtcatagtagtaattgcgcagccgcagttccactgctgcgaatccgggcctgttttccacatcgtatgtccagcacagattcatgagatcgtacatctctcttggacaccctgcagggcaccccatccgctctcctttctctaacatagcggtgacttcacttcctttcatccctcgatatggcttctgcccataggagaatgcttcccacatcaacactccaaagctccagacatcgcttttgctggagaacttgtagtagttgatgcattccggagcgtaccacttgacaggccactttccatgggtctgggccttgtagtagttttcatcagcacgcagtgctttggaaagtccgaaatcactgatcttggcgtaatgttgggtaactagcaacacatttcttgcagccagatctctgtgcacaaaattgctctcctccaagtacttcatgcccatggaaacctgatgaaccagttctatgatgttcttatccttgacatgtctgttctgctgcaaatacttattgaggggaccaagttctgccatctccataaccagcatccaggactcggcctcgcatatcccgatcatccgcacgatgtacgggttgtccagctgctgcatgacatttgcttctgctaataactcatctttaagagcggggtcattggcctcgtttttcagtattttcacagccacggttttcacaacttttttcatttggtagtagccctttttcacagttccaaaattaccagagcccagttctttgtcttccagcgtcagcagctttcggtccaggtaaacctccttgggcctgatctcctcggggtccgcgtaggggctctcgtacacctctgtgtccatgggtagggcttctctctgggggcctttgtctgcagcccagggtgcaagttctggctcatacggattgaatgacacagtactctcttgccggttcccttgggcaggggaggacgcaggatgggaacctggaagttgtggacggcctccaaaattaacatttccctgtgtgccgattttttgacatgggacagtaagaactcttaacaaaccatctgctttataagaataatgctcgactagctgccagagcgtgtcgaacttctttccctcggggatggagagcttccctgtcttgtctttgtcgatgcgatagtgcagcaccttcccttcgtgcagcaggcacagggcgtaggagccgttgttgtctctggctcggatcaggaactttccatttgtctttgatcctatcaggacaatttgctcagattcttcccgagagatttttccatggaaccaaggcattttttcatgggctgtggtagcgatcagcttctccagctgaggcttctgactgatgatggcctgctccagagcctgaccctgcaggttccatgtctgcttcacatattccctgatgaggttttccttcaaatcctcaaagggcccagtcttgggctgcaccccttggggccggttgaagggcttcttgaggaggcagaccaggccatcagactcctgggagtggtagtggcagaggtcggcggggctggcatgggtcctgccaccggcgatggcgtaggtgccattcagctcccgctcgatggtgtagtggtgtgccttcctcccgtgggccacggacagggcgaagccacccaggtagttgcggctctggcgcagcaaataaagcccatcactcatgcccccctggaccaggtaatcttctgcctcctcccgggtgatgttgccgaaaaagaagggcaggtggttggcgctgtcagccatgccgctgctggccatgcttcaggggccggagggcacacacctgcgcaggtgtccacctgcgccaggtgaggcgagggcgggcgcagcgcggggccacccgctcctcctcgctctccagccgccgccggggt

SEQ ID NO: 9279 - RNA, 4306 nt, Homo sapiens
  source 1..4306: mol_type = other RNA
agcagaggcagagaggctcaggagattgtccagggacaaggagacctggccggacctctgcagggaggtgaggcccctgcccccatcttgtcccatcacattctggatgtttggcatccccaggctcctgggaggggagaagtgctgataaaaaggccaaaaatcacacagaaagaagacagaaaactccacgcacttcctacataggtgctaccgtattcctacgagcacggggcctgtgttgaagactccctctggaagttacagaaggaagccaccaagagttcagcctcacagcctctttctcagatgcagtcaccactttaccaaacttggcacatccaaccactcctttcataattttacacctgtttgtggcctggctgacagatattttgtcattgatctttctaatttcagggattctaaatgtgttttgagaatctgctcagcactcagggattctgtctttaaaaatatgattaaaccaccagatagtgtgatttcagaaagtgtgcgtggctaccaaaaacttctaaacacaagttatatgagtgactcctgtcttctgtggctgagcttgggtactgattgtctttctccatgccttgcatcccctgttagaggagggcctgctgtccatggctgtccatgcactttaaaatgtctcaggtttagctgaagaccagatgggtccaagtttatttatatctgctggcataagaatgatggctaaattacctctttaagttgtttttttgtttgtttgttttgacagagtctcgctgtgatgcccaagctggagtgcagtggcatgatcttggctcactgcgacctccgtttcctgggttcaagcgattctcctgcctcagcctcccgagtagctgggactacagacacatgccaccatgcccggctaatttttgtatttttagtagagatggggttttaccatattggccaggctagtctcaaactccttacctcaagtgatccacccgcctcggcctcctaaagtgctgagatgtctctttaactttcaagaggtacagcaaaactgaaatcaatgggtgatgacttcttaaagatcaaacatgaagatgaggattagttaagaccagaaaatcattctccgatcttgtatcttcaactcaaattcacactccaaaaggcctgtttgtggtgaggctcagggtctttggcttgttctgaattaatactttctttggaaactctttagatggctttgatccctgtgctgccccccattgcagacacagaaagcgacaggggattctggcggcaccctctctgtggaggagaggaaggtgtggaccacgttcagaggaaggcagcctgaagctgtcctcagtgagatgctgggggatgggcctcttgcccctgctgtgcagcctccatgcagggctttatttaccagtcaccaggtcttcaagacagtctgcaggagagaggatttcagggggaaagtaagccaagccaattcattctcatggtccccttttatcacaaacatgtaagtcttccatctcataacagagacagcaaaagcagtatccaggccttttttttttttctttctttctttccttaactggctacatgcttagaaactgcactggtcaaacttgattttctttttaaagcctcaaaacatttttattgtcaggaaagcttttcagtggccagggatcagtctcatggccgtagaagcagccaaattcctctgcctttgccttcccttcaggagtcacatgctaaggcatccttgggcatttggaaaaggccgcttggggtgagagtgctctaggccactctgcaatgtccctgggcccgatgagtaacaaatgcaccccgggacccagagaagtggaaagacatgaaagggatttggaaacagatcgtaaaaataacctgtatgaaaatcacacagacaagaaaacaaacaaatccagctagccccttggatcctgccatccgtcttttctcccgggactgcctttgctttgtggagggtgagtcctgggacaggctttgggtgacaagttgtgggcatgttccatccaagcctggctctcccgactggcagagggaggtggctgacaatcaattcctctggatacattttcctgtgattgctcctgtgatcaaaggcagccaccgacaggtgcgggagcggttagttcaccacgtcatagtagtaattgcgcagccgcagttccactgctgcgaatccgggcctgttttccacatcgtatgtccagcacagattcatgagatcgtacatctctcttggacaccctgcagggcaccccatccgctctcctttctctaacatagcggtgacttcacttcctttcatccctcgatatggcttctgcccataggagaatgcttcccacatcaacactccaaagctccagacatcgcttttgctggagaacttgtagtagttgatgcattccggagcgtaccacttgacaggccactttccatgggtctgggccttgtagtagttttcatcagcacgcagtgctttggaaagtccgaaatcactgatcttggcgtaatgttgggtaactagcaacacatttcttgcagccagatctctgtgcacaaaattgctctcctccaagtacttcatgcccatggaaacctgatgaaccagttctatgatgttcttatccttgacatgtctgttctgctgcaaatacttattgaggggaccaagttctgccatctccataaccagcatccaggactcggcctcgcatatcccgatcatccgcacgatgtacgggttgtccagctgctgcatgacatttgcttctgctaataactcatctttaagagcggggtcattggcctcgtttttcagtattttcacagccacggttttcacaacttttttcatttggtagtagccctttttcacagttccaaaattaccagagcccagttctttgtcttccagcgtcagcagctttcggtccaggtaaacctccttgggcctgatctcctcggggtccgcgtaggggctctcgtacacctctgtgtccatgggtagggcttctctctgggggcctttgtctgcagcccagggtgcaagttctggctcatacggattgaatgacacagtactctcttgccggttcccttgggcaggggaggactttctgtggccaggctttgggaaggagtatgatttgattcttgagattattccacccgctgaccaagtcgcaggatgggaacctggaagttgtggacggcctccaaaattaacatttccctgtgtgccgattttttgacatgggacagtaagaactcttaacaaaccatctgctttataagaataatgctcgactagctgccagagcgtgtcgaacttctttccctcggggatggagagcttccctgtcttgtctttgtcgatgcgatagtgcagcaccttcccttcgtgcagcaggcacagggcgtaggagccgttgttgtctctggctcggatcaggaactttccatttgtctttgatcctatcaggacaatttgctcagattcttcccgagagatttttccatggaaccaaggcattttttcatgggctgtggtagcgatcagcttctccagctgaggcttctgactgatgatggcctgctccagagcctgaccctgcaggttccatgtctgcttcacatattccctgatgaggttttccttcaaatcctcaaagggcccagtcttgggctgcaccccttggggccggttgaagggcttcttgaggaggcagaccaggccatcagactcctgggagtggtagtggcagaggtcggcggggctggcatgggtcctgccaccggcgatggcgtaggtgccattcagctcccgctcgatggtgtagtggtgtgccttcctcccgtgggccacggacagggcgaagccacccaggtagttgcggctctggcgcagcaaataaagcccatcactcatgcccccctggaccaggtaatcttctgcctcctcccgggtgatgttgccgaaaaagaagggcaggtggttggcgctgtcagccatgccgctgctggccatgcttcaggggccggagggcacacacctgcgcaggtgtccacctccctttcctggattcaaacgcagatctggaatcccaggcgctgggcagtatagaatgtgggaagggaagaagcacacaaatctgagaggagtatcttaaaaggaaaacagctgaaacagagagaaagcacaagacaggcatcaacaagccagagtgct

SEQ ID NO: 9280 - RNA, 4221 nt, Homo sapiens
  source 1..4221: mol_type = other RNA
agcagaggcagagaggctcaggagattgtccagggacaaggagacctggccggacctctgcagggaggtgaggcccctgcccccatcttgtcccatcacattctggatgtttggcatccccaggctcctgggaggggagaagtgctgataaaaaggccaaaaatcacacagaaagaagacagaaaactccacgcacttcctacataggtgctaccgtattcctacgagcacggggcctgtgttgaagactccctctggaagttacagaaggaagccaccaagagttcagcctcacagcctctttctcagatgcagtcaccactttaccaaacttggcacatccaaccactcctttcataattttacacctgtttgtggcctggctgacagatattttgtcattgatctttctaatttcagggattctaaatgtgttttgagaatctgctcagcactcagggattctgtctttaaaaatatgattaaaccaccagatagtgtgatttcagaaagtgtgcgtggctaccaaaaacttctaaacacaagttatatgagtgactcctgtcttctgtggctgagcttgggtactgattgtctttctccatgccttgcatcccctgttagaggagggcctgctgtccatggctgtccatgcactttaaaatgtctcaggtttagctgaagaccagatgggtccaagtttatttatatctgctggcataagaatgatggctaaattacctctttaagttgtttttttgtttgtttgttttgacagagtctcgctgtgatgcccaagctggagtgcagtggcatgatcttggctcactgcgacctccgtttcctgggttcaagcgattctcctgcctcagcctcccgagtagctgggactacagacacatgccaccatgcccggctaatttttgtatttttagtagagatggggttttaccatattggccaggctagtctcaaactccttacctcaagtgatccacccgcctcggcctcctaaagtgctgagatgtctctttaactttcaagaggtacagcaaaactgaaatcaatgggtgatgacttcttaaagatcaaacatgaagatgaggattagttaagaccagaaaatcattctccgatcttgtatcttcaactcaaattcacactccaaaaggcctgtttgtggtgaggctcagggtctttggcttgttctgaattaatactttctttggaaactctttagatggctttgatccctgtgctgccccccattgcagacacagaaagcgacaggggattctggcggcaccctctctgtggaggagaggaaggtgtggaccacgttcagaggaaggcagcctgaagctgtcctcagtgagatgctgggggatgggcctcttgcccctgctgtgcagcctccatgcagggctttatttaccagtcaccaggtcttcaagacagtctgcaggagagaggatttcagggggaaagtaagccaagccaattcattctcatggtccccttttatcacaaacatgtaagtcttccatctcataacagagacagcaaaagcagtatccaggccttttttttttttctttctttctttccttaactggctacatgcttagaaactgcactggtcaaacttgattttctttttaaagcctcaaaacatttttattgtcaggaaagcttttcagtggccagggatcagtctcatggccgtagaagcagccaaattcctctgcctttgccttcccttcaggagtcacatgctaaggcatccttgggcatttggaaaaggccgcttggggtgagagtgctctaggccactctgcaatgtccctgggcccgatgagtaacaaatgcaccccgggacccagagaagtggaaagacatgaaagggatttggaaacagatcgtaaaaataacctgtatgaaaatcacacagacaagaaaacaaacaaatccagctagccccttggatcctgccatccgtcttttctcccgggactgcctttgctttgtggagggtgagtcctgggacaggctttgggtgacaagttgtgggcatgttccatccaagcctggctctcccgactggcagagggaggtggctgacaatcaattcctctggatacattttcctgtgattgctcctgtgatcaaaggcagccaccgacaggtgcgggagcggttagttcaccacgtcatagtagtaattgcgcagccgcagttccactgctgcgaatccgggcctgttttccacatcgtatgtccagcacagattcatgagatcgtacatctctcttggacaccctgcagggcaccccatccgctctcctttctctaacatagcggtgacttcacttcctttcatccctcgatatggcttctgcccataggagaatgcttcccacatcaacactccaaagctccagacatcgcttttgctggagaacttgtagtagttgatgcattccggagcgtaccacttgacaggccactttccatgggtctgggccttgtagtagttttcatcagcacgcagtgctttggaaagtccgaaatcactgatcttggcgtaatgttgggtaactagcaacacatttcttgcagccagatctctgtgcacaaaattgctctcctccaagtacttcatgcccatggaaacctgatgaaccagttctatgatgttcttatccttgacatgtctgttctgctgcaaatacttattgaggggaccaagttctgccatctccataaccagcatccaggactcggcctcgcatatcccgatcatccgcacgatgtacgggttgtccagctgctgcatgacatttgcttctgctaataactcatctttaagagcggggtcattggcctcgtttttcagtattttcacagccacggttttcacaacttttttcatttggtagtagccctttttcacagttccaaaattaccagagcccagttctttgtcttccagcgtcagcagctttcggtccaggtaaacctccttgggcctgatctcctcggggtccgcgtaggggctctcgtacacctctgtgtccatgggtagggcttctctctgggggcctttgtctgcagcccagggtgcaagttctggctcatacggattgaatgacacagtactctcttgccggttcccttgggcaggggaggactttctgtggccaggctttgggaaggagtatgatttgattcttgagattattccacccgctgaccaagtcgcaggatgggaacctggaagttgtggacggcctccaaaattaacatttccctgtgtgccgattttttgacatgggacagtaagaactcttaacaaaccatctgctttataagaataatgctcgactagctgccagagcgtgtcgaacttctttccctcggggatggagagcttccctgtcttgtctttgtcgatgcgatagtgcagcaccttcccttcgtgcagcaggcacagggcgtaggagccgttgttgtctctggctcggatcaggaactttccatttgtctttgatcctatcaggacaatttgctcagattcttcccgagagatttttccatggaaccaaggcattttttcatgggctgtggtagcgatcagcttctccagctgaggcttctgactgatgatggcctgctccagagcctgaccctgcaggttccatgtctgcttcacatattccctgatgaggttttccttcaaatcctcaaagggcccagtcttgggctgcaccccttggggccggttgaagggcttcttgaggaggcagaccaggccatcagactcctgggagtggtagtggcagaggtcggcggggctggcatgggtcctgccaccggcgatggcgtaggtgccattcagctcccgctcgatggtgtagtggtgtgccttcctcccgtgggccacggacagggcgaagccacccaggtagttgcggctctggcgcagcaaataaagcccatcactcatgcccccctggaccaggtaatcttctgcctcctcccgggtgatgttgccgaaaaagaagggcaggtggttggcgctgtcagccatgccgctgctggccatgcttcaggggccggagggcacacacctgcgcaggtgtccacctgcgccaggtgaggcgagggcgggcgcagcgcggggccacccgctcctcctcgctctccagccgccgccggggt

SEQ ID NO: 9281 - RNA, 23 nt, Homo sapiens
  source 1..23: mol_type = other RNA
agcagcattgtacagggctatga

SEQ ID NO: 9282 - RNA, 806 nt, Homo sapiens
  source 1..806: mol_type = other RNA
agcagcattgtacagggctatgatatacatataaatacacacacaaaattcccaataagcattcacgtcttgaacacataattttgcagtccgattccattcaaagccgtacttaagacactcagagcaaagaatcacgtttctaggagagaaggaagagttcagaacagcttagacgaatttttaaatactgatttcggcattaccatcgtcgctgtgagattaggcagagggagcggggctgaccgccagagaaccggtaccaaccaccgcaagcaatcgccgagcctcccaccccagctttcaagacaggatttacgggtacacggtgtgaacaagacaacgcaaccccctttttacaaataaaaaaaaaatcaaacaagcccccaggcccgaagacgctcatccccgccgggcaaccccgcgagcgcaggctgcgggacgaggaccttcatgctcgccgctcccgaacccccgtccgctcctgcggtcccggtgctgcggggacgtatcccgggcgctcgggtgcatggccccggccagccgaggggccgcgcgacgaccacagccggcgtggagaaggcggcgggcgccggcacttcgcggcgtccccaggcccgggctgcgccgccggggagggtcccgctctccacacctcaatggggagaagcccgcgagcgaccggccggcctctccctccatcccagagactccgcgtcgcggcgaccctccccgcgccctccacgcccccgccctcgcgtcggggagccgcctggatcccggcgcccggcgcggggccccctgag

SEQ ID NO: 9283 - RNA, 373 nt, Homo sapiens
  source 1..373: mol_type = other RNA
agcagggctggggattgcaacaccttccgagcctccctcctgccctcccttgcgccttcgagggcacaggcagccccttcctcccaggaaggagcctgtgagggaagctggtgaggcccgggcagccttcctgccttgggggtcttaaagggctggggaatgtggcaacgatgtccccctcccctgcctccggatttcctgagctcaaagctttgaggctgggcagggcccaggctcccacctggctgggtgccatccttatgccccctgccctgggggagcatcacttggaggcaggccctggctggaaggctcacccggccctaagcctcttttcagctctagccttggggaccacatcttcacagtactc

SEQ ID NO: 9284 - RNA, 406 nt, Homo sapiens
  source 1..406: mol_type = other RNA
agcaggtgcggggcggcggccgcgctggccgctcgactccgcagctgctcgttctgcttctccagcttgcgcaccagctcctgcagcttcttcacctccagctccgcgttcaccaccggcccggagcccgctccagagctgacccctgccgaggcgcatttcacctgctccgccatcatcgtgggccccgagggcgccgcggccgccggggagtgcgcgccgccgcgccggctcctcgggccacggggaggctacggctccttccctgtcgccccggcctggggggccgaccacgcgcgggctgaggccgagccggcggttcgcatcagcaccgggccctcgcctccggccgcggcagccaccaccgagctgatctgcacatgctcagtgcgtccctccagtcccc

SEQ ID NO: 9285 - RNA, 419 nt, Homo sapiens
  source 1..419: mol_type = other RNA
agcaggtgcggggcggcggccgcgctggccgctcgactccgcagctgctcgttctgcttctccagcttgcgcaccagctcctgcagcttcttcacctccagctccgcgttcaccaccggcccggagcccgctccagagctgacccctgccgaggcgcatttcacctgctccgccatcatcgtgggccccgagggcgccgcggccgccggggagtgcgcgccgccgcgccggctcctcgggccacggggaggctacggctccttccctgtcgccccggcctggggggccgaccacgcgcgggctgaggccgagccggcggttcgcatcagcaccgggccctcgcctccggccgcggcagccaccaccgagctgatctgcacatgctcagtgcgtccctccagtcccctgggcgtcgcggc

SEQ ID NO: 9286 - RNA, 4854 nt, Homo sapiens
  source 1..4854: mol_type = other RNA
agcagtgtttgttttgcccacagtacgttttaaacacggagccagcatttttaaagtttagatttctggctcctgtttaaccagctgctgtgagtagcagctgccctttaggcctgatgtctccaggtcatcccagtccccagcgtcagcggccctttctcaggcatgctgcagttgcctcatagtggacacatttctcacgtgccacctgtctcacctccctctccacaatgggagcgttaaagcacaggggctttgggtcagacgctggctcaaatcctgattctgccacctaccagctgtgtgaccttgggcatattacatgacctctgtgcctcagtttccccatctgcaaatggtgcaaagagtactcacttctcagagctgcagggactgcttgacaggacccatgccagagctctctgcacagtctggtgcaaagttaagtgctcagtaatattaagtagcattttcccctgtctggccctcataggcacttgtttgcaagtccctgatctcacaagtggccccaacactctcagacccaatgcagcgcaccttctggttttgagaaggatttttttccagcccccagaattcagaagtgaaatggtctgagtctgagggctgctctacccttactacctgtgggaccttgggggagtcactttacctctctggactcaggctgagggttttttttctgtcggctccaggggaactgacacagattggtggggcctggaaaccaacaccacagtggtgaggctactcctatggcctctaaagaatttagctgcctgtcccatccaccattgacttctttttgtagtaatgccttaggaagaggtgatcacaaccctgcaaatccagatggacatttttcagccctgggcaaccagagcatttcaccccactggccaatgtgattggttcagggatgggcacgtgacccagtccagaccaatgagagcctgccctgggacttccactgcaactactgggaatgcactttccactgagattgctgagctggtctagtaagtctcaactcaaagagaaaaacagagcttagagagaccacgttttgatgaatcatgtgagcccctgggtcctgccaaaccttaattcagaacacctgtagacttttccgttttatgagctaatacgattattttagctgtttactttaaatttctgtcatttatgagttgtcgaattctaacacccttccttgtgtggtcccctcaggcatagtcacaaatcaaaagtctagttggcaaaggaaaatggcattatgggtcacgttttaaaaaataaatgtcatggctggacgcagtggctcatgcctgtaatcccaacactttgggaggccaaggtgggtggatcacctgaagtcaagagttggagaccagcctggccaacatgctgaaaccccatctctactaaaaatacgaaaattagccgggcatggtggtgggcgcctgtaatcccagctactcagaaatgtcattatctgtgactgctctggagtcctttaggcatttccctgtccccaacaggctttcttttttctggctaatattgcagaaactatctagcctagactagctattgactatgtctgtagcgttcactacagaatcgcagtacctagttcataggagatgccttataattacttattcaacaaataaacaagttactaattggtctataatgtcctgacccggtgcagtggctcatacctaaaattccagcactttggaaggccaaggcggatcacttgaggccaggagttcaagaccaacctggacaacatagtgagaccccatttctttaaaaaaaaaaaaaaatagccaagccaggtgtggcggcatgtgctagtcccagccactcatgaggatcgtttgtgtccaggagttcaaggttgctgtgagctattacacctcacctctgcactttagcctgggtgacagagcatgaccctgtctctaaaaacatagtaataaatacaaataaataaaatgaccagcaggtccccactcacctcagcctatgagtctctgtataccaaatccatgttttcccaaccttgtcttccatttttccttagctcactctagtccagccacagtggctgcctcaccatctcttaaaatcccaagcttgttctttttttttttttctaagcgaagtctcgctcttatcccccaggtttgagtgcaatggctcgatctcggctcactgcaaccttcacctcccgggttcaaatgattctcctgcctctgcctcccaagtagctgggataaagtcgtctgccaccacgcctggctaatttttgtaaattttagtagagacagggtttcaccatgttggccaggctggtctagaactcctgacctcaggtgatctgtccgcctcagcctcccaaagtgctgggattactggcgtgagccactgtgcgtggccccaagcttgttcttgcctcagggcctgtgtacttgctgtcccatcaagaggcctcttccctcacttctttcgtgtctgacctcctctcctcccccaggtctcagctcagaggcccttcatgaccaccctgccaaagcagcaccgaccctgcttttccgctgtggttctgtcctgtttgattttcttcacaaatcaccacctgaatttccatgtgcatttatttgtttattgactcttttcccaggaggtcagctccaccaggataggtctttgttggttctttcaccgctgtacctgtgtacaggacagagcctggcacacaccaggtgccagtgaatatttgctgaaggaagtcacaaatagggatcagccatcattactttatcatcatgatcaacaggaaagaccactgtcctcacccaatcccctccaaaaggctttggagcagatgtcaacattaattcactgtctcaggtgacagctctcatcctgaggccagggttggggggagctgggaatggggcgagagtggggcctcacgtcccaggctccttgataccccccaccccacccagccaggaaacaccacgaggcagccaaggttaagtagactcttgctgctttgttataaatatattatgtacatccaaaacatgacattaaaatattactccgtgttacagaaaagatattaaggctttctattatttacattaaacaagcaagcacctttaaaaaaaaacaaaacaaaaaagccctactcttccttctctgacatactctggccagaggggataccgtgtcctcttccaaatgaccaagatgctctgcaggggctgtgccctgtgaagacatcttggtattggaaacatcagctctggcagggtgggggcagcagagaagtaggggtctagacttgagcaggaggttccagcctcttctggccggctaccctcagacccctgctgagcttcaccatccttgggggacaggctaggctgaaggtggtggctggggctgtccacctgcccagcctcccggggtcagtatgcagggctgtggcagaacaatgctccacgacgcttaggtgtgcctgggggctccccagaccactggggccagacaaggagggaaagaggcaactcactggccccaacgccagccacactgaagggctgcccagcggggcagggacggcaggcgtgcagggagtgggtaaacctcctctctaccaggggaggctggcagagtcaggcttgcagatagagcaactcaggtggctgaggaggggccgaggaaaaaaaaaaaaaagaaatgaaaaatcagtggctcaagtattctgtgtcatgaggggtgggctggggtacctgggcccagcccaggagatgtcctctccatctggaggggccagctcaaagaggctggaatttggcagatggcttcggtttgggggctagggaaggttggcaaccaggtagcaggctcggagaagttatttgatcttctgggcccatttcatgtcatctgcccgaggcttctcgcccgtcaggccctggatgaggtcctccaggcgtcgccagaagcctatcttctccagagggtagttgagccagcctgtggtgatgcagaagtaggtctcgtggggtgagacgtggtggatgcgatggtgtttacgtggcaggatgacatgccagtcctgcaggagggtgacccagcgtggcagcccaaagtacgtgtgcgaccacttgtggatctggttggtgaaggtgccgaagatgatcaggcagaagacgaagcactcccaggggtatagctgctccagggcttcagggctgtgggtgcggaacttgtaggccatgtttagcagcggcagcagtgtcaccaggcagttgtccccgttggtctcgatgaagtcgtgccgtgtgatagctgtcgggtcaatgtggtgctcccggaagggtcggatgaaagcaatgggcagctccacagagccccatgtgtcagcaccccagtgtaccaggccagacaagaagtcagcaatgagagcccctgcaacaacaccgagtatgacgaggggtgtgtcctcccagcgggccagcagcaggagatggaccaggttgtgggcgatgaggctgaagcacaggatcacagagcaccactcctggaggcgcttgcctggcgagtagagcgcagccagctcgcgggccccggcgtgctgcgcgccccagcggcaacaagacgcctcgtcctcgtccagctccagctgctggcccggccagttctcggcgcccgccatggccactcgcccgatcggcccggtgcgctctgctggcggcggcggcggcagggccgcggaaccgcggcgagatcacgccgcccaat

SEQ ID NO: 9287 - RNA, 4967 nt, Homo sapiens
  source 1..4967: mol_type = other RNA
agcagtgtttgttttgcccacagtacgttttaaacacggagccagcatttttaaagtttagatttctggctcctgtttaaccagctgctgtgagtagcagctgccctttaggcctgatgtctccaggtcatcccagtccccagcgtcagcggccctttctcaggcatgctgcagttgcctcatagtggacacatttctcacgtgccacctgtctcacctccctctccacaatgggagcgttaaagcacaggggctttgggtcagacgctggctcaaatcctgattctgccacctaccagctgtgtgaccttgggcatattacatgacctctgtgcctcagtttccccatctgcaaatggtgcaaagagtactcacttctcagagctgcagggactgcttgacaggacccatgccagagctctctgcacagtctggtgcaaagttaagtgctcagtaatattaagtagcattttcccctgtctggccctcataggcacttgtttgcaagtccctgatctcacaagtggccccaacactctcagacccaatgcagcgcaccttctggttttgagaaggatttttttccagcccccagaattcagaagtgaaatggtctgagtctgagggctgctctacccttactacctgtgggaccttgggggagtcactttacctctctggactcaggctgagggttttttttctgtcggctccaggggaactgacacagattggtggggcctggaaaccaacaccacagtggtgaggctactcctatggcctctaaagaatttagctgcctgtcccatccaccattgacttctttttgtagtaatgccttaggaagaggtgatcacaaccctgcaaatccagatggacatttttcagccctgggcaaccagagcatttcaccccactggccaatgtgattggttcagggatgggcacgtgacccagtccagaccaatgagagcctgccctgggacttccactgcaactactgggaatgcactttccactgagattgctgagctggtctagtaagtctcaactcaaagagaaaaacagagcttagagagaccacgttttgatgaatcatgtgagcccctgggtcctgccaaaccttaattcagaacacctgtagacttttccgttttatgagctaatacgattattttagctgtttactttaaatttctgtcatttatgagttgtcgaattctaacacccttccttgtgtggtcccctcaggcatagtcacaaatcaaaagtctagttggcaaaggaaaatggcattatgggtcacgttttaaaaaataaatgtcatggctggacgcagtggctcatgcctgtaatcccaacactttgggaggccaaggtgggtggatcacctgaagtcaagagttggagaccagcctggccaacatgctgaaaccccatctctactaaaaatacgaaaattagccgggcatggtggtgggcgcctgtaatcccagctactcagaaatgtcattatctgtgactgctctggagtcctttaggcatttccctgtccccaacaggctttcttttttctggctaatattgcagaaactatctagcctagactagctattgactatgtctgtagcgttcactacagaatcgcagtacctagttcataggagatgccttataattacttattcaacaaataaacaagttactaattggtctataatgtcctgacccggtgcagtggctcatacctaaaattccagcactttggaaggccaaggcggatcacttgaggccaggagttcaagaccaacctggacaacatagtgagaccccatttctttaaaaaaaaaaaaaaatagccaagccaggtgtggcggcatgtgctagtcccagccactcatgaggatcgtttgtgtccaggagttcaaggttgctgtgagctattacacctcacctctgcactttagcctgggtgacagagcatgaccctgtctctaaaaacatagtaataaatacaaataaataaaatgaccagcaggtccccactcacctcagcctatgagtctctgtataccaaatccatgttttcccaaccttgtcttccatttttccttagctcactctagtccagccacagtggctgcctcaccatctcttaaaatcccaagcttgttctttttttttttttctaagcgaagtctcgctcttatcccccaggtttgagtgcaatggctcgatctcggctcactgcaaccttcacctcccgggttcaaatgattctcctgcctctgcctcccaagtagctgggataaagtcgtctgccaccacgcctggctaatttttgtaaattttagtagagacagggtttcaccatgttggccaggctggtctagaactcctgacctcaggtgatctgtccgcctcagcctcccaaagtgctgggattactggcgtgagccactgtgcgtggccccaagcttgttcttgcctcagggcctgtgtacttgctgtcccatcaagaggcctcttccctcacttctttcgtgtctgacctcctctcctcccccaggtctcagctcagaggcccttcatgaccaccctgccaaagcagcaccgaccctgcttttccgctgtggttctgtcctgtttgattttcttcacaaatcaccacctgaatttccatgtgcatttatttgtttattgactcttttcccaggaggtcagctccaccaggataggtctttgttggttctttcaccgctgtacctgtgtacaggacagagcctggcacacaccaggtgccagtgaatatttgctgaaggaagtcacaaatagggatcagccatcattactttatcatcatgatcaacaggaaagaccactgtcctcacccaatcccctccaaaaggctttggagcagatgtcaacattaattcactgtctcaggtgacagctctcatcctgaggccagggttggggggagctgggaatggggcgagagtggggcctcacgtcccaggctccttgataccccccaccccacccagccaggaaacaccacgaggcagccaaggttaagtagactcttgctgctttgttataaatatattatgtacatccaaaacatgacattaaaatattactccgtgttacagaaaagatattaaggctttctattatttacattaaacaagcaagcacctttaaaaaaaaacaaaacaaaaaagccctactcttccttctctgacatactctggccagaggggataccgtgtcctcttccaaatgaccaagatgctctgcaggggctgtgccctgtgaagacatcttggtattggaaacatcagctctggcagggtgggggcagcagagaagtaggggtctagacttgagcaggaggttccagcctcttctggccggctaccctcagacccctgctgagcttcaccatccttgggggacaggctaggctgaaggtggtggctggggctgtccacctgcccagcctcccggggtcagtatgcagggctgtggcagaacaatgctccacgacgcttaggtgtgcctgggggctccccagaccactggggccagacaaggagggaaagaggcaactcactggccccaacgccagccacactgaagggctgcccagcggggcagggacggcaggcgtgcagggagtgggtaaacctcctctctaccaggggaggctggcagagtcaggcttgcagatagagcaactcaggtggctgaggaggggccgaggaaaaaaaaaaaaaagaaatgaaaaatcagtggctcaagtattctgtgtcatgaggggtgggctggggtacctgggcccagcccaggagatgtcctctccatctggaggggccagctcaaagaggctggaatttggcagatggcttcggtttgggggctagggaaggttggcaaccaggtagcaggctcggagaagttatttgatcttctgggcccatttcatgtcatctgcccgaggcttctcgcccgtcaggccctggatgaggtcctccaggcgtcgccagaagcctatcttctccagagggtagttgagccagcctgtggtgatgcagaagtaggtctcgtggggtgagacgtggtggatgcgatggtgtttacgtggcaggatgacatgccagtcctgcaggagggtgacccagcgtggcagcccaaagtacgtgtgcgaccacttgtggatctggttggtgaaggtgccgaagatgatcaggcagaagacgaagcactcccaggggtatagctgctccagggcttcagggctgtgggtgcggaacttgtaggccatgtttagcagcggcagcagtgtcaccaggcagttgtccccgttggtctcgatgaagtcgtgccgtgtgatagctgtcgggtcaatgtggtgctcccggaagggtcggatgaaagccttccccacaatgggcagctccacagagccccatgtgtcagcaccccagtgtaccaggccagacaagaagtcagcaatgagagcccctgcaacaacaccgagtatgacgaggggtgtgtcctcccagcgggccagcagcaggagatggaccaggttgtgggcgatgaggctgaagcacaggatcacagagcaccactcctggaggcgcttgcctccaggtctggaggagataaagggccttgattgcagatttggggcaccaggctgtctgcagactctgattcaggcatggctgttcttcagagagtgaagggcactggcgagtagagcgcagccagctcgcgggccccggcgtgctgcgcgccccagcggcaacaagacgcctcgtcctcgtccagctccagctgctggcccggccagttctcggcgcccgccatggccactcgcccgatcggcccggtgcgctctgctggcggcggcggcggcagggccgcggaaccgcggcgagatcacgccgcccaat

SEQ ID NO: 9288 - RNA, 4863 nt, Homo sapiens
  source 1..4863: mol_type = other RNA
agcagtgtttgttttgcccacagtacgttttaaacacggagccagcatttttaaagtttagatttctggctcctgtttaaccagctgctgtgagtagcagctgccctttaggcctgatgtctccaggtcatcccagtccccagcgtcagcggccctttctcaggcatgctgcagttgcctcatagtggacacatttctcacgtgccacctgtctcacctccctctccacaatgggagcgttaaagcacaggggctttgggtcagacgctggctcaaatcctgattctgccacctaccagctgtgtgaccttgggcatattacatgacctctgtgcctcagtttccccatctgcaaatggtgcaaagagtactcacttctcagagctgcagggactgcttgacaggacccatgccagagctctctgcacagtctggtgcaaagttaagtgctcagtaatattaagtagcattttcccctgtctggccctcataggcacttgtttgcaagtccctgatctcacaagtggccccaacactctcagacccaatgcagcgcaccttctggttttgagaaggatttttttccagcccccagaattcagaagtgaaatggtctgagtctgagggctgctctacccttactacctgtgggaccttgggggagtcactttacctctctggactcaggctgagggttttttttctgtcggctccaggggaactgacacagattggtggggcctggaaaccaacaccacagtggtgaggctactcctatggcctctaaagaatttagctgcctgtcccatccaccattgacttctttttgtagtaatgccttaggaagaggtgatcacaaccctgcaaatccagatggacatttttcagccctgggcaaccagagcatttcaccccactggccaatgtgattggttcagggatgggcacgtgacccagtccagaccaatgagagcctgccctgggacttccactgcaactactgggaatgcactttccactgagattgctgagctggtctagtaagtctcaactcaaagagaaaaacagagcttagagagaccacgttttgatgaatcatgtgagcccctgggtcctgccaaaccttaattcagaacacctgtagacttttccgttttatgagctaatacgattattttagctgtttactttaaatttctgtcatttatgagttgtcgaattctaacacccttccttgtgtggtcccctcaggcatagtcacaaatcaaaagtctagttggcaaaggaaaatggcattatgggtcacgttttaaaaaataaatgtcatggctggacgcagtggctcatgcctgtaatcccaacactttgggaggccaaggtgggtggatcacctgaagtcaagagttggagaccagcctggccaacatgctgaaaccccatctctactaaaaatacgaaaattagccgggcatggtggtgggcgcctgtaatcccagctactcagaaatgtcattatctgtgactgctctggagtcctttaggcatttccctgtccccaacaggctttcttttttctggctaatattgcagaaactatctagcctagactagctattgactatgtctgtagcgttcactacagaatcgcagtacctagttcataggagatgccttataattacttattcaacaaataaacaagttactaattggtctataatgtcctgacccggtgcagtggctcatacctaaaattccagcactttggaaggccaaggcggatcacttgaggccaggagttcaagaccaacctggacaacatagtgagaccccatttctttaaaaaaaaaaaaaaatagccaagccaggtgtggcggcatgtgctagtcccagccactcatgaggatcgtttgtgtccaggagttcaaggttgctgtgagctattacacctcacctctgcactttagcctgggtgacagagcatgaccctgtctctaaaaacatagtaataaatacaaataaataaaatgaccagcaggtccccactcacctcagcctatgagtctctgtataccaaatccatgttttcccaaccttgtcttccatttttccttagctcactctagtccagccacagtggctgcctcaccatctcttaaaatcccaagcttgttctttttttttttttctaagcgaagtctcgctcttatcccccaggtttgagtgcaatggctcgatctcggctcactgcaaccttcacctcccgggttcaaatgattctcctgcctctgcctcccaagtagctgggataaagtcgtctgccaccacgcctggctaatttttgtaaattttagtagagacagggtttcaccatgttggccaggctggtctagaactcctgacctcaggtgatctgtccgcctcagcctcccaaagtgctgggattactggcgtgagccactgtgcgtggccccaagcttgttcttgcctcagggcctgtgtacttgctgtcccatcaagaggcctcttccctcacttctttcgtgtctgacctcctctcctcccccaggtctcagctcagaggcccttcatgaccaccctgccaaagcagcaccgaccctgcttttccgctgtggttctgtcctgtttgattttcttcacaaatcaccacctgaatttccatgtgcatttatttgtttattgactcttttcccaggaggtcagctccaccaggataggtctttgttggttctttcaccgctgtacctgtgtacaggacagagcctggcacacaccaggtgccagtgaatatttgctgaaggaagtcacaaatagggatcagccatcattactttatcatcatgatcaacaggaaagaccactgtcctcacccaatcccctccaaaaggctttggagcagatgtcaacattaattcactgtctcaggtgacagctctcatcctgaggccagggttggggggagctgggaatggggcgagagtggggcctcacgtcccaggctccttgataccccccaccccacccagccaggaaacaccacgaggcagccaaggttaagtagactcttgctgctttgttataaatatattatgtacatccaaaacatgacattaaaatattactccgtgttacagaaaagatattaaggctttctattatttacattaaacaagcaagcacctttaaaaaaaaacaaaacaaaaaagccctactcttccttctctgacatactctggccagaggggataccgtgtcctcttccaaatgaccaagatgctctgcaggggctgtgccctgtgaagacatcttggtattggaaacatcagctctggcagggtgggggcagcagagaagtaggggtctagacttgagcaggaggttccagcctcttctggccggctaccctcagacccctgctgagcttcaccatccttgggggacaggctaggctgaaggtggtggctggggctgtccacctgcccagcctcccggggtcagtatgcagggctgtggcagaacaatgctccacgacgcttaggtgtgcctgggggctccccagaccactggggccagacaaggagggaaagaggcaactcactggccccaacgccagccacactgaagggctgcccagcggggcagggacggcaggcgtgcagggagtgggtaaacctcctctctaccaggggaggctggcagagtcaggcttgcagatagagcaactcaggtggctgaggaggggccgaggaaaaaaaaaaaaaagaaatgaaaaatcagtggctcaagtattctgtgtcatgaggggtgggctggggtacctgggcccagcccaggagatgtcctctccatctggaggggccagctcaaagaggctggaatttggcagatggcttcggtttgggggctagggaaggttggcaaccaggtagcaggctcggagaagttatttgatcttctgggcccatttcatgtcatctgcccgaggcttctcgcccgtcaggccctggatgaggtcctccaggcgtcgccagaagcctatcttctccagagggtagttgagccagcctgtggtgatgcagaagtaggtctcgtggggtgagacgtggtggatgcgatggtgtttacgtggcaggatgacatgccagtcctgcaggagggtgacccagcgtggcagcccaaagtacgtgtgcgaccacttgtggatctggttggtgaaggtgccgaagatgatcaggcagaagacgaagcactcccaggggtatagctgctccagggcttcagggctgtgggtgcggaacttgtaggccatgtttagcagcggcagcagtgtcaccaggcagttgtccccgttggtctcgatgaagtcgtgccgtgtgatagctgtcgggtcaatgtggtgctcccggaagggtcggatgaaagccttccccacaatgggcagctccacagagccccatgtgtcagcaccccagtgtaccaggccagacaagaagtcagcaatgagagcccctgcaacaacaccgagtatgacgaggggtgtgtcctcccagcgggccagcagcaggagatggaccaggttgtgggcgatgaggctgaagcacaggatcacagagcaccactcctggaggcgcttgcctggcgagtagagcgcagccagctcgcgggccccggcgtgctgcgcgccccagcggcaacaagacgcctcgtcctcgtccagctccagctgctggcccggccagttctcggcgcccgccatggccactcgcccgatcggcccggtgcgctctgctggcggcggcggcggcagggccgcggaaccgcggcgagatcacgccgcccaat

SEQ ID NO: 9289 - RNA, 70 nt, Homo sapiens
  source 1..70: mol_type = other RNA
agcatacacctgtagtcctagatactcaccctcctgagtatctaggactacaggtgtatgctaccacgct

SEQ ID NO: 9290 - RNA, 300 nt, Homo sapiens
  source 1..300: mol_type = other RNA
agcatacacctgtagtcctagatactcaggaggctgaggtgggaggatcgcagagcccgcagaggcagagttacagacggaggccagggcttaggagaaaacgtcacaggaccgcatgagcaaaccatacagtcaaactgttacttccctgtgccagaaacgagctgccggagatgcagcaaagagtaagactaatccgctgggttaggctgatggggatgcgcgaagagcaaggccctgggttaggcagagttgttgtgaggattaaagcagaatgctcgcagaggcctggcaagtcct

SEQ ID NO: 9291 - RNA, 6761 nt, Homo sapiens
  source 1..6761: mol_type = other RNA
agcatacacctgtagtcctagatatttaggaggctgaggcgggaggatcacttgagcccaggggctcgagaccagtgtgggcaacatcacaagaccctatctccaaaaaagccaaccaaacaaaaaaccggaagcagagagggtacaaaacaaatacttcaaaactcaggaatagttaggagaatttggaaataagttcatagaatgggatgagaaaacggtggctctaagtgaaagggtgagcaaatgagaatatgaaagagagtagcattgagagagacagaaacaaacattcccagggaagagtgtttctttctactaagtgggaaattcctcagatagaagcaagtctccttggttaagcaaatggatgttccatgaccaaaatgactttgttccccctaatctgcccattccactcccaatttttaaaaatttattttcatttttcctgaatacacacacagagtctagttgggaaggtgtgggcaagctctggaggggtgtgttcagagtgggtgtgtctgcggtatgagggcaggagctgatccacatgttagcagaaagggagagtcaaaaagagaaaagatatttggtcaaacttaccgacatctgccttgacctctacattctcaaatacagaaccagccagtgctacgtggtctggcagagaaagaagccatggctgcctccatgtcttgggtgcttggagcttttccatggtaccaagaggaacagtttagtgcagaactcagcctccataaaggtgagtacaagaggtgcactcagatagaatacaatcagattttatttaagttcttttttattttcctccacactggcaaaagttccgagggagcctaaagttttgtaaacattttaactatccctcttacccacccccaacttttgaatttacaaagcaaaggagagtaggagccccaacttttaatggtttcctctcccctcatgctatttgatccaaaaactatatacaattttgtagcagtctctgtatagttattacacatgtttagaagggagggaggcaagaagggatagggagaatggtgatccaaaataataaaaatagaagccaaatataatactccaaacccaaactgctctcagagcaactccagccttcttcaggcaacaatgacaggcagcaaaggtgcttttccaggggctgcccagaccacagcacctctcgcacaggcacagctgcccaatgactccaacccagtgtgagtggcaattccaggtgatgttctgtaggggtttggtggaggcaggaaaagtatttgtttataaatagggcttgagtacatttctacttgaagtttaaggttttaggaggccatgaccagaagccaggccaggcttcctgctcccattttcgcccatcccctccagcccactgcatcctcctgtatagtagattccatggatgaaggtcttaaagatggacaggttctgtatgttctcttttcagaaaaggcaaacaacttgccatcccagaatctttacacaaaaccttttccgggctacagcaagacacacacgcaatgctctgaggaccagatgaaattccaggcttttatcagaagcaaaagtttatccctatccaaaaatgaaattatacaaattcatacatatggtaaagattctagctgcctcttaaacgagacaaattttcagcagaagggcccaaaacaaaatggtcctagtcctctgaagtaaaaatatttatgggaaaaatcagtttttgtaagaaagaaaaattaagaatagtctctctcccaggccatagagcttcctttgtccaatcaggttggagcatgccaggggagatcagcttgctcagaagtcactatctaacgaagaaaaacataaatcctttcagagaaaggacactcagaaagaacaggtgaggagtgtgtaacatcaaaccaaaccaacctcatctcaaccccactcagggcctctctgatgcaatcccaaagttagcagtggcaatgcaactttcagaccgggagagctctgactgcctgttggatactcgagtcacagtccatggggtgttttgttattggccaatgtctgttaaccattaactctcttcatgattgcaccagttagaccatttgccctgatggggggaaaaagaagaagaaaaaacaaaatagaagaaaaaaagtgacaagagaaagcaagctgctaatggccgatcccaacacactttctgggagacagtagatgaaatcacagcacagtgaacacatgctgcctaaaatcagccttgttggggagtaatcccaactgccacccccaagacacagggtccagtccacttatctatagtctgagatgttcaccaacaaaaatggattaaagaatcttggacacaaagggccagaagaaaaagcctgagatgatcggttctgtgatttgttgcagagtgataaagagtaaatggtgagtaagtgttgtgtccaaaggtggagactccatagtcggcagacaggagagggatggccagtccactggcaggtgctcagtagtcatccaacgtctcgatttcacccatgttgagtcgctccgatgatgcattgactgaaaatcctaataaactgggatctgctcggaccatcttctgctttttcttcttcttgccactctgcacagcctcaaaattggattgttggttgttgctttgattggtctgaaatactgaatggagtgtactgtggttcatcccccacacagagtcctgctgttgtggctgctgtggcggctgctgtggcggctgctgctgctgctgctgtggcagctgctgctgctgacgctgctggttggctttctgtttggcacggcgctcaaggaactgcttggcaaactccttggcctcagaagtatctcctaaataggccctgatataatcatggacctcataaggagattctacttctttcaggaaagaaacaaatgtgggaacatccaagttatttgccgtattaagggcatgaagcatctgttcacaccactgcgtaaatccatcttgggctttatttactccctgaaagagcttcagcaacttttcttcttcttctactttcttattctgccggttagacacacctacagatttactgagactggcgttgtttttatttttatttgttgaattcctaggtcccacctctttcactgcatcatcccagaatcccatgttggagtttttagtgtcagcattactccaaatactactgactaggtcagatgcccactggttaggaggaccagtatttatagagccccaaacagaattcccaatgctggtgtgcaggttggaatgcgtattgttacgagctctgtttggttgctggtgttgctgctgctgctgctgctgcttttgcatttgcctggcctcttcctgctggatctccagaagagatttcgtggtacctgaaggtttgctgacattcccccaacctgagagtttctgctgttgctgttgctgctgctgctgaagagctttcatcaactccctctgctggcgcctttgctcttctcgaagctgccgttctcgttcttcctctagtttttggatttcagccaacgacagcgtggcctgggactgacatgctgttgtattggactgctggccccacgttgaagaagaaggaagcttcatctgcgccagctgttgttgctgctgctgctgctgcaacctccggagagcctcttgctgctgctgcctctggcgcattaactccttctgccgctggacctccagctcctttctcttccgttcttcttcctcatgccggagtctggctgcctcctcttccatccgcagccggttctcctctaatcgacgctgggcttcttcttcttcccgggcccattttgcagcctcctcttcctgtttgcgtaacaattcttcctgcttccgcctttcttcctcttctcttctcctctcttccagtcttctaagagcttcttcttgctgctgtctttcttcctcttctcgctgtcgccttaatgcaatttcttgctcccgctggcgacgcagagcctcttcctgtttccttcgggcaagttcttcttcctctcgccttttcctttcttcttcctgctgtcgccgaagaatttcctcctgttgtcttcggagttcttcctgcctctttcgctcttcctcttcccgttttgccctcatttctgcctctcttctctcttgctctagctttgcagctttggccttctctagctgctgaagctgttccagggcagggcctggtgtcgtggtgtccagaggaagatcccatacactaccaccttcccaaactgtaggctgtgaagctgttggctgaagctcccagatagagccagtatctggcacggacacagacctagttactgagggaatgatgttctgatcagatattctcatcttcaaggtctgaaactgttgaagaagaagtgccaactgctgctgctgctgggaagacagtgctgctttctgctgttgggccaaaacctgtgcatattgttgttgtattaaaaactgctggtactgcaggtgctgcatctggtataaggctgtgagttcttgctgcctggtcagtcgttcctggtccagctctcccatatgaggagggggagctggacctggagaaaagggaacccttccccacattttcatgatatcgccaagaggttggaagctttcatcacacgctctcttcaccaataaagacatagtaaaatagcccgcctgaaaccattctgccatctcctgattattgaagggaccttgaatttctccctgaggatctttgtaataccacttctgcattgcttcatgcatcaatggaatcgacactcctttagctctgtgctcttgcagttttgatgccaatctttcatcatctagtgcactgtcttggagataagccaccattttctcagcttgctgctccaaatgtttgagaccttcttcatcatcaggttctgtggaaacactgcccataccaggagcacctacaactggtgtttcaactggccggagagtaggactaggattgggaacaggaggtggaagtatgagaagaggagaggctgtatctgaaggaatctgcgacaggggctgctggacatcagcaaccatttcatcccctctgctgggcactttggctggtagactattttccatccgagtctcctcttcagctttttccgtttgctcagtttttggttcatctttcctctcaaactgtgatgcttcctgagactgatggtctgaaggagtacctggtctagcagatgatgatgaggtctggggagtttcctcactagcaactcctactctatctgttttctctccttctttcttatttgtcttatcgggttctttggcctcttcattatggctaccctcagagtcagagcactcctccccttcgtccacaggccggaagtccatctcctgctcttctggaataggctctttctgtactttttttagagaaaggaatgctccagatgagtcaaatgtacccatttcttcttcagcatcctctaagcaccattcgggcaagctatccctgtcatcatctatgctcccactgccagagcgaacccttcggtaaccccgttcatcatctctatctcgaaaatcaaactcaaacctccgacgtcgttccatgtgttcccgccagcctgcagaacgagggccatcaggactgtgaggtcgccacctctctccatccctccttgatccagctagtcgccaacctccatcttcatcttctccattttgttcctctctaaagatgcgccaattttcactttctgagcgtataaattcatgctttctccctactgatgttggtccaccttcctcaaaatttggtctcccttggcataaaggctgacccagcaaaagaactggtgagtacatgcaataatatccattcttctttcctacatcttttcgtcctggtttttcaaaacgtctgtcacccctttcctcccagctctgcgatctatgcatttctctgccacctcctcgaccaaaaacaccctctacttcatcaaaacttctttggtagaaaccacattcacctctgcctctgcctcgccctcttgaagaacttcgacctctaggagcccccaccactgttcctcctcctcctcgtcctgtcaatcgcaggacagcagcactatttacagacatggaaaagtttctctgttcttcttctgtaaagggtaccagagccaatggtggaaggggttcctcctggaggataggcagaaattctttatccagaaggtctgaaggtatcttgttgtctttaaggaaaagtgctaacatttcttctctgccgtaacgataatctgctaatttatacttcggcaatgctggagaaagaggaggggatgtaatactcccaccactggacagagctcggagccattcaggcccaaagttcagtgtctgcgtttccgctgccattcttttccgtatttttacaatagatttttatatgtgaagaaacctgttcaaaaattctgctggttcacagcaggagatttgagcagactttgttcagatccttttaacgctctaagagacctgggttaacaccaacataggctgtagattcaacctaatgagactggtcccactataatctgcggtccgggacagggagtctcagaaccccagtcagtcctcagcctcaacaacacaagat

SEQ ID NO: 9292 - RNA, 6544 nt, Homo sapiens
  source 1..6544: mol_type = other RNA
agcatacacctgtagtcctagatatttaggaggctgaggcgggaggatcacttgagcccaggggctcgagaccagtgtgggcaacatcacaagaccctatctccaaaaaagccaaccaaacaaaaaaccggaagcagagagggtacaaaacaaatacttcaaaactcaggaatagttaggagaatttggaaataagttcatagaatgggatgagaaaacggtggctctaagtgaaagggtgagcaaatgagaatatgaaagagagtagcattgagagagacagaaacaaacattcccagggaagagtgtttctttctactaagtgggaaattcctcagatagaagcaagtctccttggttaagcaaatggatgttccatgaccaaaatgactttgttccccctaatctgcccattccactcccaatttttaaaaatttattttcatttttcctgaatacacacacagagtctagttgggaaggtgtgggcaagctctggaggggtgtgttcagagtgggtgtgtctgcggtatgagggcaggagctgatccacatgttagcagaaagggagagtcaaaaagagaaaagatatttggtcaaacttaccgacatctgccttgacctctacattctcaaatacagaaccagccagtgctacgtggtctggcagagaaagaagccatggctgcctccatgtcttgggtgcttggagcttttccatggtaccaagaggaacagtttagtgcagaactcagcctccataaaggtgagtacaagaggtgcactcagatagaatacaatcagattttatttaagttcttttttattttcctccacactggcaaaagttccgagggagcctaaagttttgtaaacattttaactatccctcttacccacccccaacttttgaatttacaaagcaaaggagagtaggagccccaacttttaatggtttcctctcccctcatgctatttgatccaaaaactatatacaattttgtagcagtctctgtatagttattacacatgtttagaagggagggaggcaagaagggatagggagaatggtgatccaaaataataaaaatagaagccaaatataatactccaaacccaaactgctctcagagcaactccagccttcttcaggcaacaatgacaggcagcaaaggtgcttttccaggggctgcccagaccacagcacctctcgcacaggcacagctgcccaatgactccaacccagtgtgagtggcaattccaggtgatgttctgtaggggtttggtggaggcaggaaaagtatttgtttataaatagggcttgagtacatttctacttgaagtttaaggttttaggaggccatgaccagaagccaggccaggcttcctgctcccattttcgcccatcccctccagcccactgcatcctcctgtatagtagattccatggatgaaggtcttaaagatggacaggttctgtatgttctcttttcagaaaaggcaaacaacttgccatcccagaatctttacacaaaaccttttccgggctacagcaagacacacacgcaatgctctgaggaccagatgaaattccaggcttttatcagaagcaaaagtttatccctatccaaaaatgaaattatacaaattcatacatatggtaaagattctagctgcctcttaaacgagacaaattttcagcagaagggcccaaaacaaaatggtcctagtcctctgaagtaaaaatatttatgggaaaaatcagtttttgtaagaaagaaaaattaagaatagtctctctcccaggccatagagcttcctttgtccaatcaggttggagcatgccaggggagatcagcttgctcagaagtcactatctaacgaagaaaaacataaatcctttcagagaaaggacactcagaaagaacaggtgaggagtgtgtaacatcaaaccaaaccaacctcatctcaaccccactcagggcctctctgatgcaatcccaaagttagcagtggcaatgcaactttcagaccgggagagctctgactgcctgttggatactcgagtcacagtccatggggtgttttgttattggccaatgtctgttaaccattaactctcttcatgattgcaccagttagaccatttgccctgatggggggaaaaagaagaagaaaaaacaaaatagaagaaaaaaagtgacaagagaaagcaagctgctaatggccgatcccaacacactttctgggagacagtagatgaaatcacagcacagtgaacacatgctgcctaaaatcagccttgttggggagtaatcccaactgccacccccaagacacagggtccagtccacttatctatagtctgagatgttcaccaacaaaaatggattaaagaatcttggacacaaagggccagaagaaaaagcctgagatgatcggttctgtgatttgttgcagagtgataaagagtaaatggtgagtaagtgttgtgtccaaaggtggagactccatagtcggcagacaggagagggatggccagtccactggcaggtgctcagtagtcatccaacgtctcgatttcacccatgttgagtcgctccgatgatgcattgactgaaaatcctaataaactgggatctgctcggaccatcttctgctttttcttcttcttgccactctgcacagcctcaaaattggattgttggttgttgctttgattggtctgaaatactgaatggagtgtactgtggttcatcccccacacagagtcctgctgttgtggctgctgtggcggctgctgtggcggctgctgctgctgctgctgtggcagctgctgctgctgacgctgctggttggctttctgtttggcacggcgctcaaggaactgcttggcaaactccttggcctcagaagtatctcctaaataggccctgatataatcatggacctcataaggagattctacttctttcaggaaagaaacaaatgtgggaacatccaagttatttgccgtattaagggcatgaagcatctgttcacaccactgcgtaaatccatcttgggctttatttactccctgaaagagcttcagcaacttttcttcttcttctactttcttattctgccggttagacacacctacagatttactgagactggcgttgtttttatttttatttgttgaattcctaggtcccacctctttcactgcatcatcccagaatcccatgttggagtttttagtgtcagcattactccaaatactactgactaggtcagatgcccactggttaggaggaccagtatttatagagccccaaacagaattcccaatgctggtgtgcaggttggaatgcgtattgttacgagctctgtttggttgctggtgttgctgctgctgctgctgctgcttttgcatttgcctggcctcttcctgctggatctccagaagagatttcgtggtacctgaaggtttgctgacattcccccaacctgagagtttctgctgttgctgttgctgctgctgctgaagagctttcatcaactccctctgctggcgcctttgctcttctcgaagctgccgttctcgttcttcctctagtttttggatttcagccaacgacagcgtggcctgggactgacatgctgttgtattggactgctggccccacgttgaagaagaaggaagcttcatctgcgccagctgttgttgctgctgctgctgctgcaacctccggagagcctcttgctgctgctgcctctggcgcattaactccttctgccgctggacctccagctcctttctcttccgttcttcttcctcatgccggagtctggctgcctcctcttccatccgcagccggttctcctctaatcgacgctgggcttcttcttcttcccgggcccattttgcagcctcctcttcctgtttgcgtaacaattcttcctgcttccgcctttcttcctcttctcttctcctctcttccagtcttctaagagcttcttcttgctgctgtctttcttcctcttctcgctgtcgccttaatgcaatttcttgctcccgctggcgacgcagagcctcttcctgtttccttcgggcaagttcttcttcctctcgccttttcctttcttcttcctgctgtcgccgaagaatttcctcctgttgtcttcggagttcttcctgcctctttcgctcttcctcttcccgttttgccctcatttctgcctctcttctctcttgctctagctttgcagctttggccttctctagctgctgaagctgttccagggcagggcctggtgtcgtggtgtccagaggaagatcccatacactaccaccttcccaaactgtaggctgtgaagctgttggctgaagctcccagatagagccagtatctggcacggacacagacctagttactgagggaatgatgttctgatcagatattctcatcttcaaggtctgaaactgttgaagaagaagtgccaactgctgctgctgctgggaagacagtgctgctttctgctgttgggccaaaacctgtgcatattgttgttgtattaaaaactgctggtactgcaggtgctgcatctggtataaggctgtgagttcttgctgcctggtcagtcgttcctggtccagctctcccatatgaggagggggagctggacctggagaaaagggaacccttccccacattttcatgatatcgccaagaggttggaagctttcatcacacgctctcttcaccaataaagacatagtaaaatagcccgcctgaaaccattctgccatctcctgattattgaagggaccttgaatttctccctgaggatctttgtaataccacttctgcattgcttcatgcatcaatggaatcgacactcctttagctctgtgctcttgcagttttgatgccaatctttcatcatctagtgcactgtcttggagataagccaccattttctcagcttgctgctccaaatgtttgagaccttcttcatcatcaggttctgtggaaacactgcccataccaggagcacctacaactggtgtttcaactggccggagagtaggactaggattgggaacaggaggtggaagtatgagaagaggagaggctgtatctgaaggaatctgcgacaggggctgctggacatcagcaaccatttcatcccctctgctgggcactttggctggtagactattttccatccgagtctcctcttcagctttttccgtttgctcagtttttggttcatctttcctctcaaactgtgatgcttcctgagactgatggtctgaaggagtacctggtctagcagatgatgatgaggtctggggagtttcctcactagcttcaactcctactctatctgttttctctccttctttcttatttgtcttatcgggttctttggcctcttcattatggctaccctcagagtcagagcactcctccccttcgtccacaggccggaagtccatctcctgctcttctggaataggctctttctgtactttttttagagaaaggaatgctccagatgagtcaaatgtacccatttcttcttcagcatcctctaagcaccattcgggcaagctatccctgtcatcatctatgctcccactgccagagcgaacccttcggtaaccccgttcatcatctctatctcgaaaatcaaactcaaacctccgacgtcgttccatgtgttcccgccagccaggactgtgaggtcgccacctctctccatccctccttgatccagctagtcgccaacctccatcttcatcttctccattttgttcctctctaaagatgcgccaattttcactttctgagcgtataaattcatgctttctccctactgatgttggtccaccttcctcaaaatttggtctccctacatcttttcgtcctggtttttcaaaacgtctgtcacccctttcctcccagctctgcgatctatgcatttctctgccacctcctcgaccaaaaacaccctctacttcatcaaaacttctttggtagaaaccacattcacctctgcctctgcctcgccctcttgaagaacttcgacctctaggagcccccaccactgttcctcctcctcctcgtcctgtcaatcgcaggacagcagcactatttacagacatggaaaagtttctctgttcttcttctgtaaagggtaccagagccaatggtggaaggggttcctcctggaggataggcagaaattctttatccagaaggtctgaaggtatcttgttgtctttaaggaaaagtgctaacatttcttctctgccgtaacgataatctgctaatttatacttcggcaatgctggagaaagaggaggggatgtaatactcccaccactggacagagctcggagccattcaggcccaaagttcagtgtctgcgtttccgctgccattcttttccgtatttttacaatagatttttatatgtgaagaaacctgcggtccgggacagggagtctcagaaccccagtcagtcctcagcctcaacaacacaagat

SEQ ID NO: 9293 - RNA, 6768 nt, Homo sapiens
  source 1..6768: mol_type = other RNA
agcatacacctgtagtcctagatatttaggaggctgaggcgggaggatcacttgagcccaggggctcgagaccagtgtgggcaacatcacaagaccctatctccaaaaaagccaaccaaacaaaaaaccggaagcagagagggtacaaaacaaatacttcaaaactcaggaatagttaggagaatttggaaataagttcatagaatgggatgagaaaacggtggctctaagtgaaagggtgagcaaatgagaatatgaaagagagtagcattgagagagacagaaacaaacattcccagggaagagtgtttctttctactaagtgggaaattcctcagatagaagcaagtctccttggttaagcaaatggatgttccatgaccaaaatgactttgttccccctaatctgcccattccactcccaatttttaaaaatttattttcatttttcctgaatacacacacagagtctagttgggaaggtgtgggcaagctctggaggggtgtgttcagagtgggtgtgtctgcggtatgagggcaggagctgatccacatgttagcagaaagggagagtcaaaaagagaaaagatatttggtcaaacttaccgacatctgccttgacctctacattctcaaatacagaaccagccagtgctacgtggtctggcagagaaagaagccatggctgcctccatgtcttgggtgcttggagcttttccatggtaccaagaggaacagtttagtgcagaactcagcctccataaaggtgagtacaagaggtgcactcagatagaatacaatcagattttatttaagttcttttttattttcctccacactggcaaaagttccgagggagcctaaagttttgtaaacattttaactatccctcttacccacccccaacttttgaatttacaaagcaaaggagagtaggagccccaacttttaatggtttcctctcccctcatgctatttgatccaaaaactatatacaattttgtagcagtctctgtatagttattacacatgtttagaagggagggaggcaagaagggatagggagaatggtgatccaaaataataaaaatagaagccaaatataatactccaaacccaaactgctctcagagcaactccagccttcttcaggcaacaatgacaggcagcaaaggtgcttttccaggggctgcccagaccacagcacctctcgcacaggcacagctgcccaatgactccaacccagtgtgagtggcaattccaggtgatgttctgtaggggtttggtggaggcaggaaaagtatttgtttataaatagggcttgagtacatttctacttgaagtttaaggttttaggaggccatgaccagaagccaggccaggcttcctgctcccattttcgcccatcccctccagcccactgcatcctcctgtatagtagattccatggatgaaggtcttaaagatggacaggttctgtatgttctcttttcagaaaaggcaaacaacttgccatcccagaatctttacacaaaaccttttccgggctacagcaagacacacacgcaatgctctgaggaccagatgaaattccaggcttttatcagaagcaaaagtttatccctatccaaaaatgaaattatacaaattcatacatatggtaaagattctagctgcctcttaaacgagacaaattttcagcagaagggcccaaaacaaaatggtcctagtcctctgaagtaaaaatatttatgggaaaaatcagtttttgtaagaaagaaaaattaagaatagtctctctcccaggccatagagcttcctttgtccaatcaggttggagcatgccaggggagatcagcttgctcagaagtcactatctaacgaagaaaaacataaatcctttcagagaaaggacactcagaaagaacaggtgaggagtgtgtaacatcaaaccaaaccaacctcatctcaaccccactcagggcctctctgatgcaatcccaaagttagcagtggcaatgcaactttcagaccgggagagctctgactgcctgttggatactcgagtcacagtccatggggtgttttgttattggccaatgtctgttaaccattaactctcttcatgattgcaccagttagaccatttgccctgatggggggaaaaagaagaagaaaaaacaaaatagaagaaaaaaagtgacaagagaaagcaagctgctaatggccgatcccaacacactttctgggagacagtagatgaaatcacagcacagtgaacacatgctgcctaaaatcagccttgttggggagtaatcccaactgccacccccaagacacagggtccagtccacttatctatagtctgagatgttcaccaacaaaaatggattaaagaatcttggacacaaagggccagaagaaaaagcctgagatgatcggttctgtgatttgttgcagagtgataaagagtaaatggtgagtaagtgttgtgtccaaaggtggagactccatagtcggcagacaggagagggatggccagtccactggcaggtgctcagtagtcatccaacgtctcgatttcacccatgttgagtcgctccgatgatgcattgactgaaaatcctaataaactgggatctgctcggaccatcttctgctttttcttcttcttgccactctgcacagcctcaaaattggattgttggttgttgctttgattggtctgaaatactgaatggagtgtactgtggttcatcccccacacagagtcctgctgttgtggctgctgtggcggctgctgtggcggctgctgctgctgctgctgtggcagctgctgctgctgacgctgctggttggctttctgtttggcacggcgctcaaggaactgcttggcaaactccttggcctcagaagtatctcctaaataggccctgatataatcatggacctcataaggagattctacttctttcaggaaagaaacaaatgtgggaacatccaagttatttgccgtattaagggcatgaagcatctgttcacaccactgcgtaaatccatcttgggctttatttactccctgaaagagcttcagcaacttttcttcttcttctactttcttattctgccggttagacacacctacagatttactgagactggcgttgtttttatttttatttgttgaattcctaggtcccacctctttcactgcatcatcccagaatcccatgttggagtttttagtgtcagcattactccaaatactactgactaggtcagatgcccactggttaggaggaccagtatttatagagccccaaacagaattcccaatgctggtgtgcaggttggaatgcgtattgttacgagctctgtttggttgctggtgttgctgctgctgctgctgctgcttttgcatttgcctggcctcttcctgctggatctccagaagagatttcgtggtacctgaaggtttgctgacattcccccaacctgagagtttctgctgttgctgttgctgctgctgctgaagagctttcatcaactccctctgctggcgcctttgctcttctcgaagctgccgttctcgttcttcctctagtttttggatttcagccaacgacagcgtggcctgggactgacatgctgttgtattggactgctggccccacgttgaagaagaaggaagcttcatctgcgccagctgttgttgctgctgctgctgctgcaacctccggagagcctcttgctgctgctgcctctggcgcattaactccttctgccgctggacctccagctcctttctcttccgttcttcttcctcatgccggagtctggctgcctcctcttccatccgcagccggttctcctctaatcgacgctgggcttcttcttcttcccgggcccattttgcagcctcctcttcctgtttgcgtaacaattcttcctgcttccgcctttcttcctcttctcttctcctctcttccagtcttctaagagcttcttcttgctgctgtctttcttcctcttctcgctgtcgccttaatgcaatttcttgctcccgctggcgacgcagagcctcttcctgtttccttcgggcaagttcttcttcctctcgccttttcctttcttcttcctgctgtcgccgaagaatttcctcctgttgtcttcggagttcttcctgcctctttcgctcttcctcttcccgttttgccctcatttctgcctctcttctctcttgctctagctttgcagctttggccttctctagctgctgaagctgttccagggcagggcctggtgtcgtggtgtccagaggaagatcccatacactaccaccttcccaaactgtaggctgtgaagctgttggctgaagctcccagatagagccagtatctggcacggacacagacctagttactgagggaatgatgttctgatcagatattctcatcttcaaggtctgaaactgttgaagaagaagtgccaactgctgctgctgctgggaagacagtgctgctttctgctgttgggccaaaacctgtgcatattgttgttgtattaaaaactgctggtactgcaggtgctgcatctggtataaggctgtgagttcttgctgcctggtcagtcgttcctggtccagctctcccatatgaggagggggagctggacctggagaaaagggaacccttccccacattttcatgatatcgccaagaggttggaagctttcatcacacgctctcttcaccaataaagacatagtaaaatagcccgcctgaaaccattctgccatctcctgattattgaagggaccttgaatttctccctgaggatctttgtaataccacttctgcattgcttcatgcatcaatggaatcgacactcctttagctctgtgctcttgcagttttgatgccaatctttcatcatctagtgcactgtcttggagataagccaccattttctcagcttgctgctccaaatgtttgagaccttcttcatcatcaggttctgtggaaacactgcccataccaggagcacctacaactggtgtttcaactggccggagagtaggactaggattgggaacaggaggtggaagtatgagaagaggagaggctgtatctgaaggaatctgcgacaggggctgctggacatcagcaaccatttcatcccctctgctgggcactttggctggtagactattttccatccgagtctcctcttcagctttttccgtttgctcagtttttggttcatctttcctctcaaactgtgatgcttcctgagactgatggtctgaaggagtacctggtctagcagatgatgatgaggtctggggagtttcctcactagcttcaactcctactctatctgttttctctccttctttcttatttgtcttatcgggttctttggcctcttcattatggctaccctcagagtcagagcactcctccccttcgtccacaggccggaagtccatctcctgctcttctggaataggctctttctgtactttttttagagaaaggaatgctccagatgagtcaaatgtacccatttcttcttcagcatcctctaagcaccattcgggcaagctatccctgtcatcatctatgctcccactgccagagcgaacccttcggtaaccccgttcatcatctctatctcgaaaatcaaactcaaacctccgacgtcgttccatgtgttcccgccagcctgcagaacgagggccatcaggactgtgaggtcgccacctctctccatccctccttgatccagctagtcgccaacctccatcttcatcttctccattttgttcctctctaaagatgcgccaattttcactttctgagcgtataaattcatgctttctccctactgatgttggtccaccttcctcaaaatttggtctccctacatcttttcgtcctggtttttcaaaacgtctgtcacccctttcctcccagctctgcgatctatgcatttctctgccacctcctcgaccaaaaacaccctctacttcatcaaaacttctttggtagaaaccacattcacctctgcctctgcctcgccctcttgaagaacttcgacctctaggagcccccaccactgttcctcctcctcctcgtcctgtcaatcgcaggacagcagcactatttacagacatggaaaagtttctctgttcttcttctgtaaagggtaccagagccaatggtggaaggggttcctcctggaggataggcagaaattctttatccagaaggtctgaaggtatcttgttgtctttaaggaaaagtgctaacatttcttctctgccgtaacgataatctgctaatttatacttcggcaatgctggagaaagaggaggggatgtaatactcccaccactggacagagctcggagccattcaggcccaaagttcagtgtctgcgtttccgctgccattcttttccgtatttttacaatagatttttatatgtgaagaaacctgtaaatccagcgctttgggaggccaagatgggagaatcgttggagcccaggaggtggagacgtggtctctgttcaaaaattctgctggttcacagcaggagatttgagcagactttgttcagatccttttaacgctctaagagacctgggttaacaccaacataggctgtagattcaacctaatgagactggtcccactataatctgcggtccgggacagggagtctcagaaccccagtcagtcctcagcctcaacaacacaagat

SEQ ID NO: 9294 - RNA, 6628 nt, Homo sapiens
  source 1..6628: mol_type = other RNA
agcatacacctgtagtcctagatatttaggaggctgaggcgggaggatcacttgagcccaggggctcgagaccagtgtgggcaacatcacaagaccctatctccaaaaaagccaaccaaacaaaaaaccggaagcagagagggtacaaaacaaatacttcaaaactcaggaatagttaggagaatttggaaataagttcatagaatgggatgagaaaacggtggctctaagtgaaagggtgagcaaatgagaatatgaaagagagtagcattgagagagacagaaacaaacattcccagggaagagtgtttctttctactaagtgggaaattcctcagatagaagcaagtctccttggttaagcaaatggatgttccatgaccaaaatgactttgttccccctaatctgcccattccactcccaatttttaaaaatttattttcatttttcctgaatacacacacagagtctagttgggaaggtgtgggcaagctctggaggggtgtgttcagagtgggtgtgtctgcggtatgagggcaggagctgatccacatgttagcagaaagggagagtcaaaaagagaaaagatatttggtcaaacttaccgacatctgccttgacctctacattctcaaatacagaaccagccagtgctacgtggtctggcagagaaagaagccatggctgcctccatgtcttgggtgcttggagcttttccatggtaccaagaggaacagtttagtgcagaactcagcctccataaaggtgagtacaagaggtgcactcagatagaatacaatcagattttatttaagttcttttttattttcctccacactggcaaaagttccgagggagcctaaagttttgtaaacattttaactatccctcttacccacccccaacttttgaatttacaaagcaaaggagagtaggagccccaacttttaatggtttcctctcccctcatgctatttgatccaaaaactatatacaattttgtagcagtctctgtatagttattacacatgtttagaagggagggaggcaagaagggatagggagaatggtgatccaaaataataaaaatagaagccaaatataatactccaaacccaaactgctctcagagcaactccagccttcttcaggcaacaatgacaggcagcaaaggtgcttttccaggggctgcccagaccacagcacctctcgcacaggcacagctgcccaatgactccaacccagtgtgagtggcaattccaggtgatgttctgtaggggtttggtggaggcaggaaaagtatttgtttataaatagggcttgagtacatttctacttgaagtttaaggttttaggaggccatgaccagaagccaggccaggcttcctgctcccattttcgcccatcccctccagcccactgcatcctcctgtatagtagattccatggatgaaggtcttaaagatggacaggttctgtatgttctcttttcagaaaaggcaaacaacttgccatcccagaatctttacacaaaaccttttccgggctacagcaagacacacacgcaatgctctgaggaccagatgaaattccaggcttttatcagaagcaaaagtttatccctatccaaaaatgaaattatacaaattcatacatatggtaaagattctagctgcctcttaaacgagacaaattttcagcagaagggcccaaaacaaaatggtcctagtcctctgaagtaaaaatatttatgggaaaaatcagtttttgtaagaaagaaaaattaagaatagtctctctcccaggccatagagcttcctttgtccaatcaggttggagcatgccaggggagatcagcttgctcagaagtcactatctaacgaagaaaaacataaatcctttcagagaaaggacactcagaaagaacaggtgaggagtgtgtaacatcaaaccaaaccaacctcatctcaaccccactcagggcctctctgatgcaatcccaaagttagcagtggcaatgcaactttcagaccgggagagctctgactgcctgttggatactcgagtcacagtccatggggtgttttgttattggccaatgtctgttaaccattaactctcttcatgattgcaccagttagaccatttgccctgatggggggaaaaagaagaagaaaaaacaaaatagaagaaaaaaagtgacaagagaaagcaagctgctaatggccgatcccaacacactttctgggagacagtagatgaaatcacagcacagtgaacacatgctgcctaaaatcagccttgttggggagtaatcccaactgccacccccaagacacagggtccagtccacttatctatagtctgagatgttcaccaacaaaaatggattaaagaatcttggacacaaagggccagaagaaaaagcctgagatgatcggttctgtgatttgttgcagagtgataaagagtaaatggtgagtaagtgttgtgtccaaaggtggagactccatagtcggcagacaggagagggatggccagtccactggcaggtgctcagtagtcatccaacgtctcgatttcacccatgttgagtcgctccgatgatgcattgactgaaaatcctaataaactgggatctgctcggaccatcttctgctttttcttcttcttgccactctgcacagcctcaaaattggattgttggttgttgctttgattggtctgaaatactgaatggagtgtactgtggttcatcccccacacagagtcctgctgttgtggctgctgtggcggctgctgtggcggctgctgctgctgctgctgtggcagctgctgctgctgacgctgctggttggctttctgtttggcacggcgctcaaggaactgcttggcaaactccttggcctcagaagtatctcctaaataggccctgatataatcatggacctcataaggagattctacttctttcaggaaagaaacaaatgtgggaacatccaagttatttgccgtattaagggcatgaagcatctgttcacaccactgcgtaaatccatcttgggctttatttactccctgaaagagcttcagcaacttttcttcttcttctactttcttattctgccggttagacacacctacagatttactgagactggcgttgtttttatttttatttgttgaattcctaggtcccacctctttcactgcatcatcccagaatcccatgttggagtttttagtgtcagcattactccaaatactactgactaggtcagatgcccactggttaggaggaccagtatttatagagccccaaacagaattcccaatgctggtgtgcaggttggaatgcgtattgttacgagctctgtttggttgctggtgttgctgctgctgctgctgctgcttttgcatttgcctggcctcttcctgctggatctccagaagagatttcgtggtacctgaaggtttgctgacattcccccaacctgagagtttctgctgttgctgttgctgctgctgctgaagagctttcatcaactccctctgctggcgcctttgctcttctcgaagctgccgttctcgttcttcctctagtttttggatttcagccaacgacagcgtggcctgggactgacatgctgttgtattggactgctggccccacgttgaagaagaaggaagcttcatctgcgccagctgttgttgctgctgctgctgctgcaacctccggagagcctcttgctgctgctgcctctggcgcattaactccttctgccgctggacctccagctcctttctcttccgttcttcttcctcatgccggagtctggctgcctcctcttccatccgcagccggttctcctctaatcgacgctgggcttcttcttcttcccgggcccattttgcagcctcctcttcctgtttgcgtaacaattcttcctgcttccgcctttcttcctcttctcttctcctctcttccagtcttctaagagcttcttcttgctgctgtctttcttcctcttctcgctgtcgccttaatgcaatttcttgctcccgctggcgacgcagagcctcttcctgtttccttcgggcaagttcttcttcctctcgccttttcctttcttcttcctgctgtcgccgaagaatttcctcctgttgtcttcggagttcttcctgcctctttcgctcttcctcttcccgttttgccctcatttctgcctctcttctctcttgctctagctttgcagctttggccttctctagctgctgaagctgttccagggcagggcctggtgtcgtggtgtccagaggaagatcccatacactaccaccttcccaaactgtaggctgtgaagctgttggctgaagctcccagatagagccagtatctggcacggacacagacctagttactgagggaatgatgttctgatcagatattctcatcttcaaggtctgaaactgttgaagaagaagtgccaactgctgctgctgctgggaagacagtgctgctttctgctgttgggccaaaacctgtgcatattgttgttgtattaaaaactgctggtactgcaggtgctgcatctggtataaggctgtgagttcttgctgcctggtcagtcgttcctggtccagctctcccatatgaggagggggagctggacctggagaaaagggaacccttccccacattttcatgatatcgccaagaggttggaagctttcatcacacgctctcttcaccaataaagacatagtaaaatagcccgcctgaaaccattctgccatctcctgattattgaagggaccttgaatttctccctgaggatctttgtaataccacttctgcattgcttcatgcatcaatggaatcgacactcctttagctctgtgctcttgcagttttgatgccaatctttcatcatctagtgcactgtcttggagataagccaccattttctcagcttgctgctccaaatgtttgagaccttcttcatcatcaggttctgtggaaacactgcccataccaggagcacctacaactggtgtttcaactggccggagagtaggactaggattgggaacaggaggtggaagtatgagaagaggagaggctgtatctgaaggaatctgcgacaggggctgctggacatcagcaaccatttcatcccctctgctgggcactttggctggtagactattttccatccgagtctcctcttcagctttttccgtttgctcagtttttggttcatctttcctctcaaactgtgatgcttcctgagactgatggtctgaaggagtacctggtctagcagatgatgatgaggtctggggagtttcctcactagcttcaactcctactctatctgttttctctccttctttcttatttgtcttatcgggttctttggcctcttcattatggctaccctcagagtcagagcactcctccccttcgtccacaggccggaagtccatctcctgctcttctggaataggctctttctgtactttttttagagaaaggaatgctccagatgagtcaaatgtacccatttcttcttcagcatcctctaagcaccattcgggcaagctatccctgtcatcatctatgctcccactgccagagcgaacccttcggtaaccccgttcatcatctctatctcgaaaatcaaactcaaacctccgacgtcgttccatgtgttcccgccagcctgcagaacgagggccatcaggactgtgaggtcgccacctctctccatccctccttgatccagctagtcgccaacctccatcttcatcttctccattttgttcctctctaaagatgcgccaattttcactttctgagcgtataaattcatgctttctccctactgatgttggtccaccttcctcaaaatttggtctccctacatcttttcgtcctggtttttcaaaacgtctgtcacccctttcctcccagctctgcgatctatgcatttctctgccacctcctcgaccaaaaacaccctctacttcatcaaaacttctttggtagaaaccacattcacctctgcctctgcctcgccctcttgaagaacttcgacctctaggagcccccaccactgttcctcctcctcctcgtcctgtcaatcgcaggacagcagcactatttacagacatggaaaagtttctctgttcttcttctgtaaagggtaccagagccaatggtggaaggggttcctcctggaggataggcagaaattctttatccagaaggtctgaaggtatcttgttgtctttaaggaaaagtgctaacatttcttctctgccgtaacgataatctgctaatttatacttcggcaatgctggagaaagaggaggggatgtaatactcccaccactggacagagctcggagccattcaggcccaaagttcagtgtctgcgtttccgctgccattcttttccgtatttttacaatagatttttatatgtgaagaaacctgttcaaaaattctgctggttcacagcaggagatttgagcagactttgttcagatccttttaacgctgcggtccgggacagggagtctcagaaccccagtcagtcctcagcctcaacaacacaagat

SEQ ID NO: 9295 - RNA, 6415 nt, Homo sapiens
  source 1..6415: mol_type = other RNA
agcatacacctgtagtcctagatatttaggaggctgaggcgggaggatcacttgagcccaggggctcgagaccagtgtgggcaacatcacaagaccctatctccaaaaaagccaaccaaacaaaaaaccggaagcagagagggtacaaaacaaatacttcaaaactcaggaatagttaggagaatttggaaataagttcatagaatgggatgagaaaacggtggctctaagtgaaagggtgagcaaatgagaatatgaaagagagtagcattgagagagacagaaacaaacattcccagggaagagtgtttctttctactaagtgggaaattcctcagatagaagcaagtctccttggttaagcaaatggatgttccatgaccaaaatgactttgttccccctaatctgcccattccactcccaatttttaaaaatttattttcatttttcctgaatacacacacagagtctagttgggaaggtgtgggcaagctctggaggggtgtgttcagagtgggtgtgtctgcggtatgagggcaggagctgatccacatgttagcagaaagggagagtcaaaaagagaaaagatatttggtcaaacttaccgacatctgccttgacctctacattctcaaatacagaaccagccagtgctacgtggtctggcagagaaagaagccatggctgcctccatgtcttgggtgcttggagcttttccatggtaccaagaggaacagtttagtgcagaactcagcctccataaaggtgagtacaagaggtgcactcagatagaatacaatcagattttatttaagttcttttttattttcctccacactggcaaaagttccgagggagcctaaagttttgtaaacattttaactatccctcttacccacccccaacttttgaatttacaaagcaaaggagagtaggagccccaacttttaatggtttcctctcccctcatgctatttgatccaaaaactatatacaattttgtagcagtctctgtatagttattacacatgtttagaagggagggaggcaagaagggatagggagaatggtgatccaaaataataaaaatagaagccaaatataatactccaaacccaaactgctctcagagcaactccagccttcttcaggcaacaatgacaggcagcaaaggtgcttttccaggggctgcccagaccacagcacctctcgcacaggcacagctgcccaatgactccaacccagtgtgagtggcaattccaggtgatgttctgtaggggtttggtggaggcaggaaaagtatttgtttataaatagggcttgagtacatttctacttgaagtttaaggttttaggaggccatgaccagaagccaggccaggcttcctgctcccattttcgcccatcccctccagcccactgcatcctcctgtatagtagattccatggatgaaggtcttaaagatggacaggttctgtatgttctcttttcagaaaaggcaaacaacttgccatcccagaatctttacacaaaaccttttccgggctacagcaagacacacacgcaatgctctgaggaccagatgaaattccaggcttttatcagaagcaaaagtttatccctatccaaaaatgaaattatacaaattcatacatatggtaaagattctagctgcctcttaaacgagacaaattttcagcagaagggcccaaaacaaaatggtcctagtcctctgaagtaaaaatatttatgggaaaaatcagtttttgtaagaaagaaaaattaagaatagtctctctcccaggccatagagcttcctttgtccaatcaggttggagcatgccaggggagatcagcttgctcagaagtcactatctaacgaagaaaaacataaatcctttcagagaaaggacactcagaaagaacaggtgaggagtgtgtaacatcaaaccaaaccaacctcatctcaaccccactcagggcctctctgatgcaatcccaaagttagcagtggcaatgcaactttcagaccgggagagctctgactgcctgttggatactcgagtcacagtccatggggtgttttgttattggccaatgtctgttaaccattaactctcttcatgattgcaccagttagaccatttgccctgatggggggaaaaagaagaagaaaaaacaaaatagaagaaaaaaagtgacaagagaaagcaagctgctaatggccgatcccaacacactttctgggagacagtagatgaaatcacagcacagtgaacacatgctgcctaaaatcagccttgttggggagtaatcccaactgccacccccaagacacagggtccagtccacttatctatagtctgagatgttcaccaacaaaaatggattaaagaatcttggacacaaagggccagaagaaaaagcctgagatgatcggttctgtgatttgttgcagagtgataaagagtaaatggtgagtaagtgttgtgtccaaaggtggagactccatagtcggcagacaggagagggatggccagtccactggcaggtgctcagtagtcatccaacgtctcgatttcacccatgttgagtcgctccgatgatgcattgactgaaaatcctaataaactgggatctgctcggaccatcttctgctttttcttcttcttgccactctgcacagcctcaaaattggattgttggttgttgctttgattggtctgaaatactgaatggagtgtactgtggttcatcccccacacagagtcctgctgttgtggctgctgtggcggctgctgtggcggctgctgctgctgctgctgtggcagctgctgctgctgacgctgctggttggctttctgtttggcacggcgctcaaggaactgcttggcaaactccttggcctcagaagtatctcctaaataggccctgatataatcatggacctcataaggagattctacttctttcaggaaagaaacaaatgtgggaactgagactggcgttgtttttatttttatttgttgaattcctaggtcccacctctttcactgcatcatcccagaatcccatgttggagtttttagtgtcagcattactccaaatactactgactaggtcagatgcccactggttaggaggaccagtatttatagagccccaaacagaattcccaatgctggtgtgcaggttggaatgcgtattgttacgagctctgtttggttgctggtgttgctgctgctgctgctgctgcttttgcatttgcctggcctcttcctgctggatctccagaagagatttcgtggtacctgaaggtttgctgacattcccccaacctgagagtttctgctgttgctgttgctgctgctgctgaagagctttcatcaactccctctgctggcgcctttgctcttctcgaagctgccgttctcgttcttcctctagtttttggatttcagccaacgacagcgtggcctgggactgacatgctgttgtattggactgctggccccacgttgaagaagaaggaagcttcatctgcgccagctgttgttgctgctgctgctgctgcaacctccggagagcctcttgctgctgctgcctctggcgcattaactccttctgccgctggacctccagctcctttctcttccgttcttcttcctcatgccggagtctggctgcctcctcttccatccgcagccggttctcctctaatcgacgctgggcttcttcttcttcccgggcccattttgcagcctcctcttcctgtttgcgtaacaattcttcctgcttccgcctttcttcctcttctcttctcctctcttccagtcttctaagagcttcttcttgctgctgtctttcttcctcttctcgctgtcgccttaatgcaatttcttgctcccgctggcgacgcagagcctcttcctgtttccttcgggcaagttcttcttcctctcgccttttcctttcttcttcctgctgtcgccgaagaatttcctcctgttgtcttcggagttcttcctgcctctttcgctcttcctcttcccgttttgccctcatttctgcctctcttctctcttgctctagctttgcagctttggccttctctagctgctgaagctgttccagggcagggcctggtgtcgtggtgtccagaggaagatcccatacactaccaccttcccaaactgtaggctgtgaagctgttggctgaagctcccagatagagccagtatctggcacggacacagacctagttactgagggaatgatgttctgatcagatattctcatcttcaaggtctgaaactgttgaagaagaagtgccaactgctgctgctgctgggaagacagtgctgctttctgctgttgggccaaaacctgtgcatattgttgttgtattaaaaactgctggtactgcaggtgctgcatctggtataaggctgtgagttcttgctgcctggtcagtcgttcctggtccagctctcccatatgaggagggggagctggacctggagaaaagggaacccttccccacattttcatgatatcgccaagaggttggaagctttcatcacacgctctcttcaccaataaagacatagtaaaatagcccgcctgaaaccattctgccatctcctgattattgaagggaccttgaatttctccctgaggatctttgtaataccacttctgcattgcttcatgcatcaatggaatcgacactcctttagctctgtgctcttgcagttttgatgccaatctttcatcatctagtgcactgtcttggagataagccaccattttctcagcttgctgctccaaatgtttgagaccttcttcatcatcaggttctgtggaaacactgcccataccaggagcacctacaactggtgtttcaactggccggagagtaggactaggattgggaacaggaggtggaagtatgagaagaggagaggctgtatctgaaggaatctgcgacaggggctgctggacatcagcaaccatttcatcccctctgctgggcactttggctggtagactattttccatccgagtctcctcttcagctttttccgtttgctcagtttttggttcatctttcctctcaaactgtgatgcttcctgagactgatggtctgaaggagtacctggtctagcagatgatgatgaggtctggggagtttcctcactagcttcaactcctactctatctgttttctctccttctttcttatttgtcttatcgggttctttggcctcttcattatggctaccctcagagtcagagcactcctccccttcgtccacaggccggaagtccatctcctgctcttctggaataggctctttctgtactttttttagagaaaggaatgctccagatgagtcaaatgtacccatttcttcttcagcatcctctaagcaccattcgggcaagctatccctgtcatcatctatgctcccactgccagagcgaacccttcggtaaccccgttcatcatctctatctcgaaaatcaaactcaaacctccgacgtcgttccatgtgttcccgccagcctgcagaacgagggccatcaggactgtgaggtcgccacctctctccatccctccttgatccagctagtcgccaacctccatcttcatcttctccattttgttcctctctaaagatgcgccaattttcactttctgagcgtataaattcatgctttctccctactgatgttggtccaccttcctcaaaatttggtctccctacatcttttcgtcctggtttttcaaaacgtctgtcacccctttcctcccagctctgcgatctatgcatttctctgccacctcctcgaccaaaaacaccctctacttcatcaaaacttctttggtagaaaccacattcacctctgcctctgcctcgccctcttgaagaacttcgacctctaggagcccccaccactgttcctcctcctcctcgtcctgtcaatcgcaggacagcagcactatttacagacatggaaaagtttctctgttcttcttctgtaaagggtaccagagccaatggtggaaggggttcctcctggaggataggcagaaattctttatccagaaggtctgaaggtatcttgttgtctttaaggaaaagtgctaacatttcttctctgccgtaacgataatctgctaatttatacttcggcaatgctggagaaagaggaggggatgtaatactcccaccactggacagagctcggagccattcaggcccaaagttcagtgtctgcgtttccgctgccattcttttccgtatttttacaatagatttttatatgtgaagaaacctgtaaatccagcgctttgggaggccaagatgggagaatcgttggagcccaggaggtggagacgtggtct

SEQ ID NO: 9296 - RNA, 1756 nt, Homo sapiens
  source 1..1756: mol_type = other RNA
agcatgacagaggagaggtggaccccgtggtccaggggcccgggcgtggagctgacaggaagaacacagatgtcaggacgggctcagcaacacaggtcccaggtgtccggggtctcctgaactccaggaagcagtgacacccccgagggctgctgtgggtgggttcttagcttacagcaggctggccaggcagcccaggcttccggggctggttggggccgatgtactggagaggcacgtgggtaggggctgtgatccgatcagtgccgaggtaggactggagggcagggggcacgagcactgagccgtccttctgctggttactctccaggagcgcgatgagaaggcgggggacagcacaggcggtggcgttcaccgtgtgggcaaactgcagctccccagcctcggtctggaacatgatgtggaggcggcggctctggaagtctgtgcagttggaagcactggtgacctctccaaagcggcctcggcctggcatccaggcctcaatgtcaaacttgcggtaggcggggaggcccagttcttgggtgggcatatccaggacccggaagtgcaagcccagctctgtcaagatctccatctgaagggacaggaactcctccagcagctgtgagctctgctccagcccagggcctgtcaccccaaacatctccaccttggtgaagtggtgtactcgatacagcccccggggttcctgtcccgtgtttgtctctgcccggtagcaggtgctggagcaaaccatcctgactggcaggtccctgaaggccacggtgtggtccatgaagtagcctgcaagccccacctccgctgttccagccaggttgagatctttgaagcgggcagggtcgatgttgtaaatttgggatgggttggcatttggtgtcatcccacagccttcaaacactgctccgcggagaaggtctggcaccgtcatgggggtgaagccccggcggagaagcttgttgaatgtgaagttgaccaggccgtgctgcaggagggctccagccccgcgcaggtaataggaccggtggccagacacgtgggacaggcgcttctgacggatgatgtcgagtttctcgccaatttccaggtggccccgaggttggaaggagaaaactggcttgtctccgaccatgtggagcactcgagcctggctctcatccccgacgggcacgtctgggtgggtctggttgggcagcttcagcgcctgcaggtagaactgctcctcaagctgggcctccacaaggagagaaagctggcctgggaatgggaggaacgtaggaccaaatatggagccagcacctggatccagccgcacctgctgcacttcaccactgtcctggtttgccagcagggcccgcactgcctcagtcacagctgccttctcttcctccaggctccggatctgctcctgcagctgcctcagctcctgccatgtcgagatgatcgcgggcaggtccgccgagcgcagctcccccttgcggagctccagggcgtgtgcggcctcttctgggcatgcgcagaaccgctctatgtccagctgagggagtgcgctgtagccctcgcgcgcatactcgtacaggaggttccggtttcgtttctctgtagtgaaacttctccttggactatcgttggagatgcagcctccccggggccggaacccccgacgagtcagcaaaggccacaagcgccgcgccatggacgcagccatcttggaccgggaacaaggcggcacttc

SEQ ID NO: 9297 - RNA, 1750 nt, Homo sapiens
  source 1..1750: mol_type = other RNA
agcatgacagaggagaggtggaccccgtggtccaggggcccgggcgtggagctgacaggaagaacacagatgtcaggacgggctcagcaacacaggtcccaggtgtccggggtctcctgaactccaggaagcagtgacacccccgagggctgctgtgggtgggttcttagcttacagcaggctggccaggcagcccaggcttccggggctggttggggccgatgtactggagaggcacgtgggtaggggctgtgatccgatcagtgccgaggtaggactggagggcagggggcacgagcactgagccgtccttctgctggttactctccaggagcgcgatgagaaggcgggggacagcacaggcggtggcgttcaccgtgtgggcaaactgcagctccccagcctcggtctggaacatgatgtggaggcggcggctctggaagtctgtgcagttggaagcactggtgacctctccaaagcggcctcggcctggcatccaggcctcaatgtcaaacttgcggtaggcggggaggcccagttcttgggtgggcatatccaggacccggaagtgcaagcccagctctgtcaagatctccatctgaagggacaggaactcctccagcagctgtgagctctgctccagcccagggcctgtcaccccaaacatctccaccttggtgaagtggtgtactcgatacagcccccggggttcctgtcccgtgtttgtctctgcccggtagcaggtgctggagcaaaccatcctgactggcaggtccctgaaggccacggtgtggtccatgaagtagcctgcaagccccacctccgctgttccagccaggttgagatctttgaagcgggcagggtcgatgttgtaaatttgggatgggttggcatttggtgtcatcccacagccttcaaacactgctccgcggagaaggtctggcaccgtcatgggggtgaagccccggcggagaagcttgttgaatgtgaagttgaccaggccgtgctgcaggagggctccagccccgcgcaggtaataggaccggtggccagacacgtgggacaggcgcttctgacggatgatgtcgagtttctcgccaatttccaggtggccccgaggttggaaggagaaaactggcttgtctccgaccatgtggagcactcgagcctggctctcatccccgacgggcacgtctgggtgggtctggttgggcagcttcagcgcctgcaggtagaactgctcctcaagctgggcctccctggggtacaggtgaacaagctccttccggatctcccggccacgtgcccgcagaccctggtacttggggtcctgctgcacttcaccactgtcctggtttgccagcagggcccgcactgcctcagtcacagctgccttctcttcctccaggctccggatctgctcctgcagctgcctcagctcctgccatgtcgagatgatcgcgggcaggtccgccgagcgcagctcccccttgcggagctccagggcgtgtgcggcctcttctgggcatgcgcagaaccgctctatgtccagctgagggagtgcgctgtagccctcgcgcgcatactcgtacaggaggttccggtttcgtttctctgtagtgaaacttctccttggactatcgttggagatgcagcctccccggggccggaacccccgacgagtcagcaaaggccacaagcgccgcgccatggacgcagccatcttggaccgggaacaaggcggcacttc

SEQ ID NO: 9298 - RNA, 1042 nt, Homo sapiens
  source 1..1042: mol_type = other RNA
agcatgacagaggagaggtggaggacgtctggtgctgaactttagaggcatgagcagtactaactgtgcttgtcttcatggtggccttattcacagtaacagcccggtgcctccggttatgtgggggggtggtactgacagcagcactttgaggcatacttaatctattcacgggtgttgggggagcactgtctgatcggggtctagaaatacctaagaatgcatccaccagacagctgattccacgcatggcacgaaaaaatatttgaggcagatgtttaaggcagggatactgattcaattcttgcggcattccgctcacattcaagaactgttcctgaaatttgggagtagagcttataatagctgggttactcaaatccacaggattacttaacatgtgtaaaaagcgaaaccatgtctgtgcaacacactcattatccatttctggagggatcagactggcatcttcatcgggaactttaaatgcaggaaatgaaggaccatatgtaaagcgtagcaatctggaagtgagtgcacaaatgaccttgctccactgctccaccactgctgggtgatgcctccagttagccaccatctccttggctgttttccaataaggaggtgttgggaagcaccgagtacaagctagtaaccacacctcaaagagaacaccaatcaacttctctgctagattctcagcaatgccaccttgaacagttggtggggccagaagtatgtcgttaatctgcagaagaaacaacagtaagacttcccaagtttctcgggccatgagagatgactcacgggccagtttctgaatggctctcaggacctgtaagcatagtcgaatctgactggaaccctgttcctgtctgttcctcaggtactgaggctccttcctcctcattcagaaggcctaaattcagaggcagggtccaaagttctaaagcttggtacaaaaagattctgtaggtgttttagtatagtttgaacatattgattaggctctttaataactggcaatggaatagaatctttt

SEQ ID NO: 9299 - RNA, 1581 nt, Homo sapiens
  source 1..1581: mol_type = other RNA
agcatgacagaggagaggtggaggacgtctggtgctgaactttagaggcatgagcagtactaactgtgcttgtcttcatggtggccttattcacagtaacagcccggtgcctccggttatgtgggggggtggtactgacagcagcactttgaggcatacttaatctattcacgggtgttgggggagcactgtctgatcggggtctagaaatacctaagaatgcatccaccagacagctgattccacgcatggcacgaaaaaatatttgaggcagatgtttaaggcagggatactgattcaattcttgcggcattccgctcacattcaagaactgttcctgaaatttgggagtagagcttataatagctgggttactcaaatccacaggattacttaacatgtgtaaaaagcgaaaccatgtctgtgcaacacactcattatccatttctggagggatcagactggcatcttcatcgggaactttaaatgcaggaaatgaaggaccatatgtaaagcgtagcaatctggaagtgagtgcacaaatgaccttgctccactgctccaccactgctgggtgatgcctccagttagccaccatctccttggctgttttccaataaggaggtgttgggaagcaccgagtacaagctagtaaccacacctcaaagagaacaccaatcaacttctctgctagattctcagcaatgccaccttgaacagttggtggggccagaagtatgtcgttaatctgcagaagaaacaacagtaagacttcccaagtttctcgggccatgagagatgactcacgggccagtttctgaatggctctcaggacctgtaagcatagtcgaatctgactggaaccctgttcctgtctgttcctcaggtactgaggctccttcctcctcattcagaaggcctaaattcagaggcagggtccaaagttctaaagcttggtacaaaaagattctgtaggtgttttagtatagtttgaacatattgattaggctctttaataactggcaatggaatagaatcttttggcaacactaaagccataatccagtctgtatatacatcaacgcaatattttacagtctctccatccaatggaagggtcagtccatagcaaattacttccatggtccattttacttctttgtcagtttttaacaaattctcactaccagccactgaaggggtacctaacacctgcccaagaggacggactacagcatttgccacctctcgtccaacgctctctggatagctgtgcagcacactggtatggccttgatcattctgaatcaccaaatgcagtgacctccactcagagtacatcgtgccactaaagtacaatccaaatggcacctgaggcgacgggcggggcccgcatcgccggggcgggcgccgccgccggccgtcctcggccttccgcctcacgcgacccgcgccatagggctggcgctttcaccgccctggccggccgtcctcaggcggtccgtcagtccacccgtcagcgactctcccagggcgccaagggacgacgaaggccactcgagccagccggctgggatctgc

SEQ ID NO: 9300 - RNA, 1379 nt, Homo sapiens
  source 1..1379: mol_type = other RNA
agcatgacagaggagaggtggaggacgtctggtgctgaactttagaggcatgagcagtactaactgtgcttgtcttcatggtggccttattcacagtaacagcccggtgcctccggttatgtgggggggtggtactgacagcagcactttgaggcatacttaatctattcacgggtgttgggggagcactgtctgatcggggtctagaaatacctaagaatgcatccaccagacagctgattccacgcatggcacgaaaaaatatttgaggcagatgtttaaggcagggatactgattcaattcttgcggcattccgctcacattcaagaactgttcctgaaatttgggagtagagcttataatagctgggttactcaaatccacaggattacttaacatgtgtaaaaagcgaaaccatgtctgtgcaacacactcattatccatttctggagggatcagactggcatcttcatcgggaactttaaatgcaggaaatgaaggaccatatgtaaagcgtagcaatctggaagtgagtgcacaaatgaccttgctccactgctccaccactgctgggtgatgcctccagttagccaccatctccttggctgttttccaataaggaggtgttgggaagcaccgagtacaagctagtaaccacacctcaaagagaacaccaatcaacttctctgctagattctcagcaatgccaccttgaacagttggtggggccagaagtatgtcgttaatctgcagaagaaacaacagtaagacttcccaagtttctcgggccatgagagatgactcacgggccagtttctgaatggctctcaggacctgtaagcatagtcgaatctgactggaaccctgttcctgtcttggtacaaaaagattctgtaggtgttttagtatagtttgaacatattgattaggctctttaataactggcaatggaatagaatcttttggcaacactaaagccataatccagtctgtatatacatcaacgcaatattttacagtctctccatccaatggaagggtcagtccatagcaaattacttccatggtccattttacttctttgtcagtttttaacaaattctcactaccagccactgaaggggtacctaacacctgcccaagaggacggactacagcatttgccacctctcgtccaacgctctctggatagctgtgcagcacactggtatggccttgatcattctgaatcaccaaatgcagtgacctccactcagagtacatcgtgccactaaagtacaatccaaatggcacccgtcagcgactctcccagggcgccaagggacgacgaaggccactcgagccagccggctgggatctgctcaggcaacttccgact

SEQ ID NO: 9301 - RNA, 1521 nt, Homo sapiens
  source 1..1521: mol_type = other RNA
agcatgacagaggagaggtggaggacgtctggtgctgaactttagaggcatgagcagtactaactgtgcttgtcttcatggtggccttattcacagtaacagcccggtgcctccggttatgtgggggggtggtactgacagcagcactttgaggcatacttaatctattcacgggtgttgggggagcactgtctgatcggggtctagaaatacctaagaatgcatccaccagacagctgattccacgcatggcacgaaaaaatatttgaggcagatgtttaaggcagggatactgattcaattcttgcggcattccgctcacattcaagaactgttcctgaaatttgggagtagagcttataatagctgggttactcaaatccacaggattacttaacatgtgtaaaaagcgaaaccatgtctgtgcaacacactcattatccatttctggagggatcagactggcatcttcatcgggaactttaaatgcaggaaatgaaggaccatatgtaaagcgtagcaatctggaagtgagtgcacaaatgaccttgctccactgctccaccactgctgggtgatgcctccagttagccaccatctccttggctgttttccaataaggaggtgttgggaagcaccgagtacaagctagtaaccacacctcaaagagaacaccaatcaacttctctgctagattctcagcaatgccaccttgaacagttggtggggccagaagtatgtcgttaatctgcagaagaaacaacagtaagacttcccaagtttctcgggccatgagagatgactcacgggccagtttctgaatggctctcaggacctgtaagcatagtcgaatctgactggaaccctgttcctgtcttggtacaaaaagattctgtaggtgttttagtatagtttgaacatattgattaggctctttaataactggcaatggaatagaatcttttggcaacactaaagccataatccagtctgtatatacatcaacgcaatattttacagtctctccatccaatggaagggtcagtccatagcaaattacttccatggtccattttacttctttgtcagtttttaacaaattctcactaccagccactgaaggggtacctaacacctgcccaagaggacggactacagcatttgccacctctcgtccaacgctctctggatagctgtgcagcacactggtatggccttgatcattctgaatcaccaaatgcagtgacctccactcagagtacatcgtgccactaaagtacaatccaaatggcacctgaggcgacgggcggggcccgcatcgccggggcgggcgccgccgccggccgtcctcggccttccgcctcacgcgacccgcgccatagggctggcgctttcaccgccctggccggccgtcctcaggcggtccgtcagtccacccgtcagcgactctcccagggcgccaagggacgacgaaggccactcgagccagccggctgggatctgctcaggcaacttccgact

SEQ ID NO: 9302 - RNA, 1544 nt, Homo sapiens
  source 1..1544: mol_type = other RNA
agcatgacagaggagaggtggaggacgtctggtgctgaactttagaggcatgagcagtactaactgtgcttgtcttcatggtggccttattcacagtaacagcccggtgcctccggttatgtgggggggtggtactgacagcagcactttgaggcatacttaatctattcacgggtgttgggggagcactgtctgatcggggtctagaaatacctaagaatgcatccaccagacagctgattccacgcatggcacgaaaaaatatttgaggcagatgtttaaggcagggatactgattcaattcttgcggcattccgctcacattcaagaactgttcctgaaatttgggagtagagcttataatagctgggttactcaaatccacaggattacttaacatgtgtaaaaagcgaaaccatgtctgtgcaacacactcattatccatttctggagggatcagactggcatcttcatcgggaactttaaatgcaggaaatgaaggaccatatgtaaagcgtagcaatctggaagtgagtgcacaaatgaccttgctccactgctccaccactgctgggtgatgcctccagttagccaccatctccttggctgttttccaataaggaggtgttgggaagcaccgagtacaagctagtaaccacacctcaaagagaacaccaatcaacttctctgctagattctcagcaatgccaccttgaacagttggtggggccagaagtatgtcgttaatctgcagaagaaacaacagtaagacttcccaagtttctcgggccatgagagatgactcacgggccagtttctgaatggctctcaggacctgtaagcatagtcgaatctgactggaaccctgttcctgtcttggtacaaaaagattctgtaggtgttttagtatagtttgaacatattgattaggctctttaataactggcaatggaatagaatcttttggcaacactaaagccataatccagtctgtatatacatcaacgcaatattttacagtctctccatccaatggaagggtcagtccatagcaaattacttccatggtccattttacttctttgtcagtttttaacaaattctcactaccagccactgaaggggtacctaacacctgcccaagaggacggactacagcatttgccacctctcgtccaacgctctctggatagctgtgcagcacactggtatggccttgatcattctgaatcaccaaatgcagtgacctccactcagagtacatcgtgccactaaagtacaatccaaatggcacctgaggcgacgggcggggcccgcatcgccggggcgggcgccgccgccggccgtcctcggccttccgcctcacgcgacccgcgccatagggctggcgctttcaccgccctggccggccgtcctcaggcggtccgtcagtccacccgtcagcgactctcccagggcgccaagggacgacgaaggccactcgagccagccggctgggatctgctcaggcaacttccgactgccaggggcggcggcgtcaaata

SEQ ID NO: 9303 - RNA, 1093 nt, Homo sapiens
  source 1..1093: mol_type = other RNA
agccaggctctgaagggaaagtttgccagatgcattactagtgtcagcaaaattgaaagaagcatttttcagtcaattatgaaagtaaactgttctcaaacaatcttagcagaaatgctaatttacatacaattgatatgtcacaatcagatttcatctattgctaacatattaccccccagccaataaaagtagtttcttagaagctcccaggagagaagcctctagttcttttactgtgtatatttgaaagtaataaaggcttatttctttagaagtgctttcttaatcagacttttccttagtttagccagaacttcacagaaaattagtcttttgctagcgaggcttcctgttacatgaggttttccatttgaacacacgggtgttagtgcaagaaacatcctgtctttcatgtcattcaagtgactgatgaatgtgaaggggcttcttcctcaagtcttctaggtagacagcagaaagcacaataccgagtagccaatcctctcttctctcatttctcaaggtggcttttaaggttgaaaaaaatccttccttaattttccttgttcttttattctccaaattttctgatttttatttccagatacacacttcccctgaaatccaggtccaatattatagatccaagcagatctgagacaccttcagcaccgactgggcaatccaggtttcctagaggcgaggcctaggacccaactgtccccaaattgctttactcccagttcctgggtgggtccagtcctcatgtctgggcttctctttcgggggcccaattcagtggcctgctcagtcttcctacaggtctgattgccctaccttgaactacaatacatctgtttgagatctggtttttgtcttcatctttcctaggtcagatcctgtctgctggttgaagttaggtcatatgtctgctgaactgtcagagcaccttgacttctgaatgtgtcttttgtctaatttttcctctgctgttctgaacccaggcaaccagacctcctggtagggactaaatcacattgaacaactgcacctggacatacccaattgtctccccaggacagggttttga

SEQ ID NO: 9304 - RNA, 202 nt, Homo sapiens
  source 1..202: mol_type = other RNA
agcccctgcccaccgcacactggaacagttgacccatgtgaggagcaaacgttttagaaatctcggaaccccctccaaaggagaggaggtgctctgagccttccggaagggcctctctcttccaaggacacaccagcagaggaggagggtgcagagaagctgtgagggctgtgagtgctcctggaggcacacagcttttacc

SEQ ID NO: 9305 - RNA, 340 nt, Homo sapiens
  source 1..340: mol_type = other RNA
agcccctgcccaccgcacactggaacagttgacccatgtgaggagcaaacgttttagaaatctcggaaccccctccaaaggagaggaggtgctctgagccttccggaagggcctctctcttccaaggacacaccagcagaggaggagggtgcagagaagctgtgagggctgtgagtgctcctggaggcacacagcttttaccaaacacttccagctaagctcctgcccatactgccccatcccctcccctcctcccttcctggctctctcttccccttccttcttatcctgttagctcctgcgccagctgctggagctggggtttctgctgaatcaccac

SEQ ID NO: 9306 - RNA, 1301 nt, Homo sapiens
  source 1..1301: mol_type = other RNA
agcccctgcccaccgcacactggaacagttgacccatgtgaggagcaataagcagatggcagccaggagccgaaggccagactctggggggaagcaggtggggaagagcggctgcagcacgtagttggagaaggtgagggcgatgacagcctggttggtggggtagatcaccagcacagcaatccacagcctcaggaacccagccagtcctccgaagatgtccttgacataggagtagtcacctccagatttggggatggtgaccccgagttcagcatagcagagggctcccacaactgtgatgaagcccgtcacaatccagacgatgagagcaaggcccacagaaccagcattctccagcactccctttggcgagacaaagattccagagccgatgatgttccctacgatgataccacaggcactgaccaatccgatctctttcttcagggctactccgccccctccggaaccagcctcggggctggcgtccgactcgcccccacctgggtgtttcttttcggtgttgtttcggtgcctggctccttcttccatccttctcagtaggattgcaacctcaaaagctgcctccctttctaaatgcgtattcgtgtaaatatattgggagagagctttgaattagaacgtccttttccgaaataggaaccactgctactctctaaaaaaggcaagcagataaaagagaacacgaaaaatattcctactccgcattcacactttctggtcactcgcgtttacaaacaagaaaagtgttgctaaaaaaaaaaaaaaaaaaaaaggccaggggagacatacatttaaatataaaaatagaactgtgccagcgactccggctggaattctgctgaaagggatgtgtcttcagaaaccaggatggttctgctctgtgcaccaggcagtggcttattcagaaagtgagcctggatttcccttcacctctccccctaataaaacaggagactgcctttacctccccttagttttttcttttatgatgaagacaaaagtagttttcattaacggtaggaaaaaagagcaatcctcaggtactttcttctcttctagaaaaacaaactgtgaacctgacggtgttgctctagatctggtttccacctgctttgggtttcttttcccttccccgtcttctgcttccgcctttcccaggtgtcctcttctttctcgctggtcttcgtgcccttgttttcctcttttcgatccccgttctactgcacagccggccccatccctctggtttcgggagagtggcttctccacacact

SEQ ID NO: 9307 - RNA, 182 nt, Homo sapiens
  source 1..182: mol_type = other RNA
agcccctgcccaccgcacactggaacagttgacccatgtgaggagcacttttgctggggcgttcacttctctgccttctgccacgctctggccagctcccacagactccctcccctccagctggagcaaaaggggtgaggcatgtccctcccagcagccctctgggtctgggtgcccaggct

SEQ ID NO: 9308 - RNA, 1631 nt, Homo sapiens
  source 1..1631: mol_type = other RNA
agccgcggggatcgccgagggccggtcggccgccccgggtgccgcgcggtgccgccggcggcggtgaggccccgcgcgtgtgtcccggccgcggtcggccgcgctcgaggggtccccgtggcgtccccttccccgccggccgcctttctcgcgccttccccgtcgccccggcctcgcccgtggtctctcgtcttctcccggcccgctcttccgaaccgggtcggcgcgtcccccgggtgcgcctcgcttcccgggcctgccgcggcccttccccgaggcgtccgtcccgggcgtcggcgtcggggagagcccgtcctccccgcgtggcgtcgccccgttcggcgcgcgcgtgcgcccgagcgcggcccggtggtccctgccggacaggcgttcgtgcgacgtgtggcgtgggtcgacctccgccttgccggtcgctcgccctttccccgggtcggggggtggggcccgggccggggcctcggccccggtcgcggtcccccgtcccgggcgggggcgggcgcgccggccggcctcggtcggccctcccttggccgtcgtgtggcgtgtgccacccctgcgcccgcgcccgccggcggggctcggagccgggcttcggccgggccccgggccctcgaccggaccggtgcgcgggcgctgcggccgcacggcgcgactgtccccgggccgggcaccgcggtccgcctctcgctcgccgcccggacgtcggggccgccccgcggggcgggcggagcgccgtccccgcctcgccgccgcccgcgggcgccggccgcgcgcgcgcgcgcgtggccgccggtccctcccggccgccgggcgcgggtcgggccgtccgcctcctcgcgggcgggcgcgacgaagaagcgtcgcgggtctgtggcgcggggccccggtggtcgtgtcgcgtggggggcgggtggttggggcgtccggttcgccgcgccccgccccggccccaccggtcccggccgccgcccccgcgcccgctcgctccctcccgtccgcccgtccgcggcccgtccgtccgtccgtcgtcctcctcgcttgcggggcgccgggcccgtcctcgcgaggccccccggccggccgtccggccgcgtcggggcctcgccgcgctctaccttacctacctggttgatcggttctcggcggcgtcgcggcgggtctgggggggtctcggtgccctcctccccgccggggcccgtcgtccggccccgccgcgccggctccccgtcttcggggccggccggattcccgtcgcctccgccgcgccgctccgcgccgccgggcacggccccgctcgctctccccggccttcccgctagggcgtctcgagggtcgggggccggacgccggtcccctcccccgcctcctcgtccgcccccccgccgtccaggtacccggcggccgtcgcgcgcctgccgcgcgtgtggcgtgcgccccgcgccgtgggggcgggaacccccgggcgcctgtggggtggtgtccgcgctcgcccccgcgtgggcggcgcgcgcctccccgtggtgtgaaaccttccgacccctctccggagtccggtcccgtttgctgtctcgtctggccggcctgaggcaaccccctctcctattgatcat

SEQ ID NO: 9309 - RNA, 77 nt, Homo sapiens
  source 1..77: mol_type = other RNA
agccttccaggagaaatggagagacggagactgggagagaccccaagcgcgcgagaaataaagccaggggcggccag

SEQ ID NO: 9310 - RNA, 9314 nt, Homo sapiens
  source 1..9314: mol_type = other RNA
agccttccaggagaaatggagattctctctccactagaatctcatgctgaaggaggctggtgcgggcttgttcacaaagtggcagtcttccaagagggtgaggggcaaactctgaggccaattgaggtagaggcttggaagttacacagcatctcttcctgtgcattctgcttcaaagcaagtcaagagcccagcccagattcaaaggatagggaaatagactcatgtcttaatgggaggggcttccaggaatttgtggccatatttaatccactgtagagtggttattctcattacgaaacattctttattacaacatttagtatggctgtaccttaagtagagcctcctggaatagatttaaaaggttgctcaactggtaagacccacaaatggagagctgccactgctttccttagttctttgtctgaccaccagatggtggcattgctcagtcgaccccgagtatttcaaggccggcaccaaattccacctggagatgcccttcaagctgtgggaattctatgattttgcacagctggattgggagcaggcagtgctacctatggagagggtctgggattagggttgcaatgggcattggatgcctctttctccctgactcttctagaactgttgtgggaaatttcttcacctccccaaatgggggactggagtaagatgctgcaaatatcatcccatcacaatggactcaatcatgaagaaaaatatcgtttgtaataaaaaaattgtttgcatactcatgaattgtctatcgaaattacattgtattgatttcatcctagtgatgtaaataattctataccacttctttttcttttttctaccctctgcaccattatagttgtttgtataacagtgtctgcaaaaactgataacatttgattaaggcctgcagtctagtccattgtattgtgccagtgtcaatttcctggttttgatcatgtaatatagtgatataagatgttatcattggggaagataggagataaggacatagacctttctgtactatttttgcaacttcttgcaagtctataagtatttcagaatagaaagttaaaaaaataccctcactaaaaataacctccacctgcttgtgtattactggtatttgcatcatcatttgggagaaaagttgagcattgattttaaaaactctttttttgggggggggggtcattctggcagggtagcactggcttctcaacccccttcagatccactggccacttccacagatcctgcccaggctcaaagcacctgctagactaggtgatcagtggtgcagagacctggagccaaggatggggagagacagtcattgccacctcctttcttccctttctggactcagagatcctctgtcccaagtttctcccttatagtcagggctctgccctttactactcactttcttgtttgttgtcttaatcgtgggttacaatgcttctctaagactaacaggaagacacttttatttccattttgtgaataagaaaactaacacccagggtttgaggtacttggctgggaccaaaagtaagtgatgcatccaaggctagaaggtagattaaatgactttttaatctgggttttccttgctaatttctaaatacactaaaaagagaaaactttttagaaagttttctttctgaaagagaaagccttttagaaagttttctttctgaaagagaaaactttttagaaagttttctttctgcaagagaaagccttttagaaagttttctttctgaaagagaaaactttttagaaagttttctttctgaaagagaaaactttttcaagtgaagtaaaacttctttgaaatattacgtgtttaaactcctaggctgtaatttcatatgcttttatttactgtcttgttctattaaaatgcaacctatagcaccttttaatgttcacacagtgtttgaagtagagaaatgaaacttttatgagtaagtggagaaagtagtgttaactttttttttcattaatgagaaaacaataggcagcaatgggtttaggagttctatggcgaaaaggcatttcctgagattgaatcagtggcaaaaggagagcctgttatgttttgctaaccaaaagaatgtgggaacattttagctaaaatgcaagttaaaactgtgaaacatataaataagcatttggtatgcttttcagtttccacaacagtagtcaagccagtgagccctgtggggagggctcatgggccctggactcaaagagctcagagtatgtctacctggggaactaaaccagtgtgcatgaaatgaccagagagtgatatggggcagatagggtttcatgccagggtgtgtaccatggttgtgtctggaaacaagggctaccgaggcctggatcactcagaggaggcatcagggagaatgtactggacttgggctcaatgtagagatgtagggggtagctctcttttgactcctaaaattacagtgaaaaactgggttctcgtaatcacacttacgagttgttgtgtccctggactagttatatcttctctctctctctctctttctctctctctcgctctctgtgtgtgtgacaaaatactcataccacaaaatttaccattttgattattttaaggtacacagttcagtgccactaagtgcatttacaatgctgggcaatcatcatgactatttagttccaggaccttttcattacccacaaaggagaccatgtgcccattaagcagtcactctctccttggcaaccacttaatgtggttttcgtctttatggacttgcctactgtgtgacacacagtgttttgtggtggatgggaaaatgtatgatatttaggccttactctcaaggagcttactaattgggaagatgtaatctgagaacatgaaaaagacagttacatcctatgaccaacatcatgcttgctgggaaaaccttagaagcattcccaattacagtcagaaataagataagagatgctaaatgtcaccgctgtgattcagcattgtgctgaagaacctagccaatgcagtaagacaagaaaaataaatgaagcacaaggatggaaagtaagagacaaattattgttatgtggagatgatatggttgtgtactttcaacgagttgcttacctcttttattatatgtaatacttttggaaattcagtgtccatgtacagaaagcaatagcatttctgccgaactacagtaacctataggaaatgttatagaaaaaaagatacagttcacaataacaataaaacaatagggtacctagaaaaaaattaaataaaatatgcctagttctttaatagaaaaaattataaaacataaagtatatcataagtagaatatgatatgttcgtagataggatagctcatttgtgtaaaagtgtctcattgaagacaattccaataaatatcccaacaggatttatcttgcaattacagaaaccaattctaaaattgatttgaagagtaaggtacatccacaggtctgatatgtctaaaaaagaataaaagggtcaagaaagcaaatgaaagagcagagaaacaggcctaagaatcactgtgaatttaatactagataacagtgcatgatgaatgagtgggaaaggctgagcacatcattgacttatcttgagacaactagctttctataaaaaaagatactagatctgcatctcacaacacataccaagataaatctcagctaaaccagcatgtgaaaatcaaaatgttaacactgtcagaagccaaccccgggagaatatctttatgacctgagaggttaaaaagaattccttagaaaggatccaaaaaacacaactcagaagtgaaaaaaatgataaatttgactaggttaaagtattatgatttataggtgtataatataagattatggcctagaagtatacacataggtgttgcctctggacacagagtgaggggagagaatgggacaggggacatcagctttatccatcatgtgaaaaatgataaaaatgttaacattggttaatcctggttggtggggacacaagggcttgttacacttagaaatatttccatgtttaaaaaatttttaagacaacacaaagcaactaccaacctcagcatgaaaggtggaaactatcgttgtatagggggaaattgccaaacccaaaatcctgattgatcttatcactgccatcagcaagctgcgtccatgggtgaggaccttcctctcaggggctgtgtgctcattgtgttccagttgcctccagcattcagtacaggaacatgctgtgcaagtttgtagcctaggagcaatagggtatatcatatagcctaggtgtgtatgtacactctatgatgttcgcatgacaaaattgcctaacaacacatttctcaagacatgtctctattgttaagcagcacatgactgtatatataacaatggtttctttaaaagcactcccaggagtggccaggtgcagaaatagctgaatttgtgagcaatgataatgatagttaatataattatcatattttccagagcacctgcacatcacgtttgatctttacagtgagtggaacagacattacgatctccatttgacagatgaggaaattaaaccttagagttatcagatttcaaaggtgaagggaccttagagatcctttcatccagctttctcattttacaaaaaaaagaactccctgagatccagggaaactaactgacctaggatcccacagggagtgaataagggctgttgggccaggcccaggtcttctgatttctagcttcctgattttgcactccattgcgctattctcagtcttcagtgtgttagaggaaacttggtaggttatgcatttgttcttaaggagaaattttgttgatatcagtcctaggcactattttataaatgcacacatgtggaaaaatcccttattttcctgctttttttctatatatagatacaggcagatacacagacagatagacacaccacatgtggatgtcactggggagatgaaggtgggattgaacttagcagagtctcaaagggggcttcagctttatctgtcaaatattcttttattaaaaaattttgaagcaaaatgaccattacagtagcatttattcattttggataatgggcactgaattcataagtgtttgttttcctcttcatatttctgtattttaaaattttcaaaaaaaaccaaatatggatattaaaaataaattctcacctataataccataccctcattttataaaaataaagaatattttcaaagaaataaaaatggttcagaaggatggaaagaaaactatactatgggactcgttagttaagttgacattaatcctctgctttaagtctttcctgtgatgacactagcagaatgtgtatcattttctctgcatttgctgcaggatcagttctctttggcaggttttgagccgttctaataagtccagcatgaaaggcaggcctctcgtgtcagttctaaacccaccagctgccccattgtgactgcatagtcccctggttctgagactgtgctctgcctgataagcgacgtacggagcacagtggactgaaagcccggggatctgataccaaacatgttagttaaactcatgtttaactaacccaaactcatgtttaactggcccaaaggaagtaggcccagaaatgtggtttttggagctccctttaatgaacgtgtaaacagaggatagaatattggccttacagtttaaaaaccctccttcaagtcccagtcaagtcccttattcactggatgacctcacacggttcatctgatctttcttggtctcagtcttcttactatagactggaaatggtcatatttgacttagctgtccatatggctgttctggagatgagacagctaatgaagtgagaacactcattaacacaccaactgaaaaacacaaaacaaaagagagatgataggattatattgctgttatgaatcattccaagaggtgtcatggtgatatgaatcatcatatggtaatgtcatggctaaggcccaaacacagaatagcagcattgacccagtagtctcgaaattagtcacagaggccaagctagtgaagacccagcagccctattgttatcaagaaagagcactatccaaaaggtgtgtggcctcatcttctccttgcaaagagagaattcatctggtatatgttgataggcgtgtatccgaccacagctacctccatcagccctgaggacagaggcagcctgcattccagtcccagctcttctctgtctcggtgtgtgacttaggcggtttcacagaggacgccaacttcattggcttttgcggttttttgtttgtttgttttttgttgttttctttttgtttgttttgttttgtttttgtctgtagaatgagtgagttaaactaaattgtctgtaaggcctcagctcactcttaaagtgtgatcactagctagagtttgaactttagccccaatatgactgttgtgttgtcattgtcacctttgtaacctgacattcaggaatgtccctctctagttcatattctgacctagcttctgaaagcattatagcagagttgagaatttttgatctaggaaagataaatattaaaaagaaattcccaccaaaataccataaataaggaatgttttaaagaaaaatggttcagaaggaaggaaaactataatgtagttcttgttagttaagttgacattaatcctctctttgctttaagtctctcctgtgttgacactagcagaatgtgtcataaagacatggaaagatcataaattctcaactctgctctaaagatctgaccttcagcgttgcatttatttggccacacctttatagtgtggtcatacctagaaaatattttcttgcctggtcatcagccctctcacctcgattactttctatattttagcacaaaagaagaaatggcgcattcaccactcagccagttgcactggaagtgaatttaaattcctgaactggttatcttggaagatattgtgcttattgcagatgtggccggtgcatgagtttaggcactaccatgctctgggctgtggttcttggctcctgcttctggatggctggacattaccaggagagagcctgctgatacatctacgcacattcactctactgcacttcagctgtgtccttgttattccacagccctttaagtcctggttcaccaaccagatgttaagactctcttggatccctcaaatcccatccccatgcctgctgcctcctctctcagcagttgcccactccttatcttctaatcctcttttctccctatgatgatgatagtgaccctgtagctccaactactgggtcctcacagtcagtccactcctgcagaggaaactggagggtgaccaggaaccttcaagtcaatgtgggccacagacaggaaccgtctttaaaagatggttaaatgcccgtggtttacgtaggttggctttctttaagcaaataaaggaaatgcattgcttcatgtccagcaaagtacagggtggattcaggagaagctggctcaaggcattcctaggaagtcatcaaggagctgcctgtacctctgtcttcaggccagcatcttctgagttggctttattctcaagcaggctgtcattaagtgatggcttaacaacaatttagcaaccatggcatgacagagaatcatgcctgatagctctaacaaagtatccgagagtgttcccccatgagccaatcactgttgccagagggatgtggttcttggactggccaggtctgagacacgttgcttgggcccctatttgtgcagaattggcccctgactacattcccagagggtctttggatgtttggtcagatggtctgtactctggggggatcaattcataccagcaaggtccagtcagcccctacacctaccaccgcctctctagtggaagccacttttgcatctaattgtcttgggaattgtgttggttttctattgctgctgtaacaaattgccacaaatttaatggcttataataacatacatgtattatcttacagttctggaggccataagtccaaaaccagcctcactggactacggtcaaggtgttagttccttctggaggctctaagggacaatctgtttcctggtcttttctagtttctaagaggcttcctgcatttctttggctcatggccccttcctccatcttcaaagccagcagcaaagcatcttctctcctctctgacttctgtttccatccttatatcttctcgctgactctgatcctcctgcttccgtcttagaaggactcttgtgattacattgggcataccaaattaaattcagaaattcagataatcaagatctttaattcaatcatgtctgcaaagtcccctttaccatgtaagataacatattcacagcctctgtgggttagaatgtgaacatttttattattcagcctactgcagggattatccactcaatttaaaaacctgaacttagacagagaaagagtgtactgaagctcctgcattggagtgggaaattgtagatagtgacctaggaaggtgactttgtacctgcttgtaggtttagttttatttgcttcttgggtgtatttagattgtcctttttgagctgtttgtgggtttttctccacagaattgggtactcataaaagaggtgtccatattgcctcaaagccaccagattctgatgagccataccccttatcttccttcttcattttgttcacggcaattactttgtgcccataaagtgggaggcagtgtgctgaggaaatacaagattctccaagacacactcctttctcttgtggaacttatgtctggtggagtagaaaggcacgcacgcaattatttttaacccaaggcacaggatgtgctgagtgatataaaagtgacaaactaaggagtgggaagacagcaggagacatcagttccagcttccaggggtgtcagatcatgcaccccaatttttggttcagaaatatgatcactactatatgcacctcaatttcaggttattaactattgcaggctaagaattttagggctttaaaaatagtatgatgtgttttttcttctttgtctagggtgtttggatgaaagcaggtgctcagctctgatgattcatgtgaaatcacttctactcaaggttgactaaagttgggaatgatgaaaatttcctagtcaaagcaaaaattaagaagaaaac

SEQ ID NO: 9311 - RNA, 706 nt, Homo sapiens
  source 1..706: mol_type = other RNA
agcgtgggatgtccatgaagtcagaaaaatggctgttctttttcacatctgggacattatgagttttcttcgtgtgagcagcccaacccactatcccaatgtccaatggaaacacaacttctttgtcagggcccaccaggttgtcctcaaacttggaggtgggggtgacatccagcaacctagaggccacctcaggtatgccgttccgggaccggcacaggaacatgctgcagcggtcagcctggagcaggtgggccagcctctgcagggccctgtgaaccccctgctctggggtgcccccctcctcctgcacggtccacagcagctccaagcacagggctgactcctccacctgggtcagctcagagaaggacatgctggactggactggcacctggctgttcttgaagatttctcccagcacctccacccgcaacttcctgtcaaagtactccttggcaaactgagggttctcctccaggtatttctccacggcaacttggttgatctcacccatggtgtggcttgctttgctgcgtttgttcagaaaggacgaccttcagagcactacctgaggcagagtgatgagaaggaaattcatcctggtggaaattactgaggaaaccgtaaatggtccctcataggacttccaaaggtcaagcagaaagcagagctttcaaactgcctgtaactcttgggatgtgac

SEQ ID NO: 9312 - RNA, 25 nt, Homo sapiens
  source 1..25: mol_type = other RNA
agctacagttacttttgcaccaacc

SEQ ID NO: 9313 - RNA, 3173 nt, Homo sapiens
  source 1..3173: mol_type = other RNA
agctacagttacttttgcaccaacctaacaaaatatggttcaaaataaaagtctgaatttcctattgtttttggaaaatcaggtttgacaaccctatgttgattccaccatctctctcctcatgtcctgggagaggattttgcctcagtgatcacaaatacaagtgaacagtgaaggccatttccacctgactcaacagaaatgttggctggatcacaaaggctgtatcaatggcctagacctcccttctctatccttgttttcctgcctgcatagcaatgaccttgaggtgaaaatcccagaggctacaggattccataaaatttctgacaatgacctcagctacacaagatacacaattctgtaggtcctgaggatttctgtacctgctcatccttaagagccataataacgaacatcatggaaacctctgtaaaaggggcacattctatttattgcagtgttattgcagttttccactctctatcaatccagtacttctataacaattataattcctactataatcttaccacctgtggtgctaccctgtggaattcaggatatcaaggcatacaggacctggggaacagatttcccccactggcactgaacacgatgcagtattccttgtgaacaagagaacaatttcatgttgctttcagaaacatcaaaggatgtcaagtaactgctgcctcctcaggctgacctctatggcatccaggatataaattaggacaataccctgtagttttttctcagaggccttgaatagcaatgaaaactaggctcaaactagagagagagctatattctgccatcctactgtccctgtccctgtccctgttgagctacacaatgtttgggatctccaaaaaaagttattcaccccttcatgttagcagaacccaactgttttcaaaccaacccatacatatagaacccccaagattaataaggcctttgttattgtacaaaccaaggcaataagaggcagttggttcccacagttggtgatttgaaggctggcaaactctatcaagagtcatgtgagaccaacaatatcctgaaatatgtagtccctcttttcaggtcaccagcagagtcctctgggccaaactgggtcaggtccatggcctaactcatcagaaaggaaaaaaaaaaaacggaataaatgcttaggctatttacaaattcctcccatgaacagaacaccaaggttcacttacctgaatacactgggatgggtgagtggtgcacactggtggtcacctgccaggcagtagaggtaaaatggcttccactatagtatcagcagagacataaatctgacatgggccctgggcagggcaaaaggtgcaatgcagttcacacatacctggaatttatgcagatgttcagatataggatgttcaattcaggctgatgccaccctcataagggatctccttcagagctgttatatcaactggacatccctacatatcaaaagtgtctttcccttgtgaactgtgtggcactcaatgagatatggccttcagctgaagctttctgacattcactgtgtactcaaggactttctccagggtgctaacagattttccacatttgccactcataaggcttttatcgactatgaattctctgatgtttaataaggctggagttatggctaaaggatttcccacattccgtgcactcataaggcttctccccagtgtgaaccctcctgtgcttaatgaggccggaattttgagtaaaggatttcccacattcactgcactcatagggtcttgatccagtgtgaactctctggtgttttcggagactggagctgtagggaaagaacttcccacattcactgcactcataaggcctctccccagtgtgaactccccgatgttgaaggagtgcagacctttggctaaaggatttcccacattcgctgcacttataaggcctttctccagtgtgaaccctatggtgttcaatgaggctagagttttggctaaatgacttcccacattcgctgcactcataaggcctggatccactgtgaactttctggtgttttatgagactggaatgatatgtaaaaaacttcccacattcactgcactcataaggcctctccccagtgtgaactccccgatgttgaaggagtgcagacctttggctaaaggatttcccacattcactgcactcatatggcctttccccagtgtgaactctccgatgtttaatgaggttagacttgttgctaaataattttccacattcatcacattcatgaggtcgtactgcagtgtgaactctccggtgctgaatgagactagagctttgcctaaaggacttcccacactctcgacattcataaggcttttctccagtgtgaagtctccaatggtcattgagactgtagcttttgctaaaggatttcccacattcactgcatatgtaacatctttctgtagtgagggttctctgctgctgaacaagtgtgtgtttaccgctgaatgcttttgtgtgttctccacagttgtaatgagtttttcctctgtgactgatggccccaccgtcgcttttgctatttgattgctccccagtgtgagcagcctgttgatggagaaatcccaacttggccaggaagtccttcccaacttctctgcaggtggaaggctcccctgacacatggaatgtgcaggtcttcacaaacaaggctctgcccacattgcttctgaaatgtttttctccaaggtgctgcttctgatgatgaacatctagagaggttaaaagagccaagttctccagcatcacatcacggtacaggcatctttgagcctcatcaaggagaccccattcctcccaggagaagtgtacggccacatcttcaaaggtcacagtgccctgagttggcgtcctcagagtggccgctgccatcagactctgcgggtagagctgggccgggagcgacgggcgacattggtagggacccggggacagcggtccctatcccaggcctgacgtgggtcccccagggcggcgtcgccaaggcttagacgctttcgtgcaggagggacgacgactcccctcacgccttcgtggccccaactcggcgctctgctatctctgatccggtgaacacacctcagagaagctaaaatggccgccac

SEQ ID NO: 9314 - RNA, 3081 nt, Homo sapiens
  source 1..3081: mol_type = other RNA
agctacagttacttttgcaccaacctaacaaaatatggttcaaaataaaagtctgaatttcctattgtttttggaaaatcaggtttgacaaccctatgttgattccaccatctctctcctcatgtcctgggagaggattttgcctcagtgatcacaaatacaagtgaacagtgaaggccatttccacctgactcaacagaaatgttggctggatcacaaaggctgtatcaatggcctagacctcccttctctatccttgttttcctgcctgcatagcaatgaccttgaggtgaaaatcccagaggctacaggattccataaaatttctgacaatgacctcagctacacaagatacacaattctgtaggtcctgaggatttctgtacctgctcatccttaagagccataataacgaacatcatggaaacctctgtaaaaggggcacattctatttattgcagtgttattgcagttttccactctctatcaatccagtacttctataacaattataattcctactataatcttaccacctgtggtgctaccctgtggaattcaggatatcaaggcatacaggacctggggaacagatttcccccactggcactgaacacgatgcagtattccttgtgaacaagagaacaatttcatgttgctttcagaaacatcaaaggatgtcaagtaactgctgcctcctcaggctgacctctatggcatccaggatataaattaggacaataccctgtagttttttctcagaggccttgaatagcaatgaaaactaggctcaaactagagagagagctatattctgccatcctactgtccctgtccctgtccctgttgagctacacaatgtttgggatctccaaaaaaagttattcaccccttcatgttagcagaacccaactgttttcaaaccaacccatacatatagaacccccaagattaataaggcctttgttattgtacaaaccaaggcaataagaggcagttggttcccacagttggtgatttgaaggctggcaaactctatcaagagtcatgtgagaccaacaatatcctgaaatatgtagtccctcttttcaggtcaccagcagagtcctctgggccaaactgggtcaggtccatggcctgaatacactgggatgggtgagtggtgcacactggtggtcacctgccaggcagtagaggtaaaatggcttccactatagtatcagcagagacataaatctgacatgggccctgggcagggcaaaaggtgcaatgcagttcacacatacctggaatttatgcagatgttcagatataggatgttcaattcaggctgatgccaccctcataagggatctccttcagagctgttatatcaactggacatccctacatatcaaaagtgtctttcccttgtgaactgtgtggcactcaatgagatatggccttcagctgaagctttctgacattcactgtgtactcaaggactttctccagggtgctaacagattttccacatttgccactcataaggcttttatcgactatgaattctctgatgtttaataaggctggagttatggctaaaggatttcccacattccgtgcactcataaggcttctccccagtgtgaaccctcctgtgcttaatgaggccggaattttgagtaaaggatttcccacattcactgcactcatagggtcttgatccagtgtgaactctctggtgttttcggagactggagctgtagggaaagaacttcccacattcactgcactcataaggcctctccccagtgtgaactccccgatgttgaaggagtgcagacctttggctaaaggatttcccacattcgctgcacttataaggcctttctccagtgtgaaccctatggtgttcaatgaggctagagttttggctaaatgacttcccacattcgctgcactcataaggcctggatccactgtgaactttctggtgttttatgagactggaatgatatgtaaaaaacttcccacattcactgcactcataaggcctctccccagtgtgaactccccgatgttgaaggagtgcagacctttggctaaaggatttcccacattcactgcactcatatggcctttccccagtgtgaactctccgatgtttaatgaggttagacttgttgctaaataattttccacattcatcacattcatgaggtcgtactgcagtgtgaactctccggtgctgaatgagactagagctttgcctaaaggacttcccacactctcgacattcataaggcttttctccagtgtgaagtctccaatggtcattgagactgtagcttttgctaaaggatttcccacattcactgcatatgtaacatctttctgtagtgagggttctctgctgctgaacaagtgtgtgtttaccgctgaatgcttttgtgtgttctccacagttgtaatgagtttttcctctgtgactgatggccccaccgtcgcttttgctatttgattgctccccagtgtgagcagcctgttgatggagaaatcccaacttggccaggaagtccttcccaacttctctgcaggtggaaggctcccctgacacatggaatgtgcaggtcttcacaaacaaggctctgcccacattgcttctgaaatgtttttctccaaggtgctgcttctgatgatgaacatctagagaggttaaaagagccaagttctccagcatcacatcacggtacaggcatctttgagcctcatcaaggagaccccattcctcccaggagaagtgtacggccacatcttcaaaggtcacagtgccctgagttggcgtcctcagagtggccgctgccatcagactctgcgggtagagctgggccgggagcgacgggcgacattggtagggacccggggacagcggtccctatcccaggcctgacgtgggtcccccagggcggcgtcgccaaggcttagacgctttcgtgcaggagggacgacgactcccctcacgccttcgtggccccaactcggcgctctgctatctctgatccggtgaacacacctcagagaagctaaaatggccgccac

SEQ ID NO: 9315 - RNA, 1056 nt, Homo sapiens
  source 1..1056: mol_type = other RNA
agctacagttacttttgcaccaacctaataaaaccatgattaaaaaaataataaacatttaaaaagcggtggggggagtggggcgcgggggcgagccggagaagcaggcgtcagtgtttgctaaagaaaccaaggcccagaagagagttaaatgttttgcccaaggtcaggcaaagagttggcaggaggtctagaggagaattcaggcttcctcatctaaactccaagcttttccgcccaagcagggcatgccctggggccaacccctccaggaagcctgggtagtgtccttccctgcatttccccagtggctgctgcctcaaggtgactcagaaggaagctgttgtctctagttcctcctcaccaatccagctggtcttaggatcgggaaaaagataagctaattgtctggtggttaattaactccagccaactaatgatctgaacttgccgcggatacccagccagcggaagtgcggttaactgcccgagggatgccccgaacaccggccgagccaacttccggccgcagaggctgccgggcaggggttatggcggccgccagagtgagccagcttggtgtccggggacacttggggcactgcggatggacagcgctggttttcaataccagggacctaagtccgggtggggagcggcccctcagcgccccagacccctgccacggtgccggtgacgggccacgcccaaaatatcaggaaaagcgtctcagtcctccttgtgggcggagaagagacccagcggccgagcccgggggcctcagatccccagctgctcattggcctgtgtctgtcgccccccggtggccgcgtgagggactggagcccggctttgctcctcccgttggcctcgtttctcttcctggctttgcgtgtcccgaccactaaaagccccaaacatgacgaagtaaaatgggcaccgtcaaaaaccgcatttgaagacagtgcgcatgagcgcatggttaagttttcagacgttttgcaagctggatgttaaatacattttttgacgtcattgttaaaaaataaattttat

SEQ ID NO: 9316 - RNA, 381 nt, Homo sapiens
  source 1..381: mol_type = other RNA
agctacagttacttttgcaccaacctaatacaaaccatcccatatctgtgttctccatcctttcatcctttatcacagtggggttgtgatagatccctgaaaacacaggatcaagtataggtaaatgcaagatggtacatagaatcaagtgtgaaagtgagtcccatcaacccacactctttccatttggcccagttgctgcccttgttgtttagaatggcacgtacctggccttgaaatgcactgaagcctatggggattactttaaaattcggtcctgtaagccagtctgttagtatcattgctcctactaatgatagaaattgctggtgttggccgggtgtggtggctcacaccagtaatccaagcactttggcagac

SEQ ID NO: 9317 - RNA, 4638 nt, Homo sapiens
  source 1..4638: mol_type = other RNA
agctacagttacttttgcaccaacctaatatttcacagccactctcctggatgtttctggggagcttcagtctaggctcagacatggtgcctgctggttctgggaaaaggttaaggggctgagtagtagcacacactacatcctccagactgtctatgccatggctatgtttggaaaccctgcaaatggcctggcagagtctcaccttgccaatccagagaggatgtgggggatttctggcttaagaataggctgaaaagagggactggaggttactgccacatagccaagcattcctgggaactttctgggaatgtgaactgatatgaaaatggcttagactacaagaattatagggaaatatcagaatacccacctaaaaatggcttaaataagaaggccattttaaagcttacttcatgaggaattttgaaataggcagttccagggtcagtttggctgctcaacagagtcttcaaggacggaggcactcttcataattctcttctgccatcatcaggattcagtgaaatctccctctatggtcacaggatgactccagcagttctgattatcctgggttcagcaataactgcgttggttctcgtttcctcagtctttccctcttcttggaggatgagagccagaagtcacccaacttgtactggtatctgaacaggacactgaagattatgtttacatttgtttgactgactgttgtctcaggttgctgtgtctcctggggatggctctgtgtggtccacccaaagctgaacagctgctttagatctttattgttgtcgtagcagtggagactgtgtaggttggtagcctcagagcaacaggctataccatccagcctaggcgtatagtaggctattccatctcaatttgtgtaagtacattccatgatgttcataaaacaacaaaatcacccacaatgcatttctcagaatgtatccttattgttaagtgacaaatgactgtatatagttttaactaaataaagttacctggagctcagtccctgagaacatgtctcctgtttaaacaagaatagaaagatgttaaaggcctactagtactaaactgaaatttttctccttgatactaggaaattaaaaggggaaacactttgtctctacctgatttagagtgtttaatgtaccattaccacctaaaatgatgtcccagattactagttgaagcattccatacattgggaaatactagattaaagaaacaaagagaaaggatcaaatagcctcactcactctcccattcattcatttctcttgttatgggcctgaaactgggtatgtagtgttgaacaacaaaaaccaaattcctgcccccattgacttaaccattgaacacggatcttttcttccttgtaacctattctatcatgcatctactcttgctctgtcaaattcttttcatcccagctcttatctcattgctgtcccaatatagtgtaactcatttggaggactagaaattccttgaagttcttgttctcctctgacatcagaccagtccctatgtgtaaggccaagccttggaatgtgcctggaaggctctgtctctggttcacaggctagatctccaagcctctagcaaatttggacaatacgtcatatctctcatgtctttcctgaaattcctgcatgatcagagaagttggggaggcaggggggtatatctaataataagaggtccaggatcatgattattctttcttttgtgctactatttagtgacaagttaggttttaatccaaaagtgtgctctggggcctcaagtacaaaatcaggctgcctcaattgtcttaacattgcctggtagaatcccttaaatgaggggtggttaatgcaaaatatatgtattttattaatatattatttggtatattagtaagtgcttttttaggtttccatataaaatctttcctccaatgttattaccaagcctcagaacttcttcagagttaatgcctgtgaactcctcatttaatgccccattgttctcacagaaattaattacagcgaatgttgtctgacttcatgggagtttaatgacagagattatgacctcacattccctttgcagaaggaaagcaggtgtggccaagaccggctttactaaaagcctcccactacatctttattcgaagaaatatagttatctatagttagaacttggaacttccaaattgtatttgttgttctgactgaacttttgtcaaattatataagtgcttcgataaggagttgtatctctcccattacccttctaaatttagaaatgataatttttgacatcctctaggggaagaaaattcttgaaagctctgataaaagcaaatttgttaacaaatttaaaaggtaatgttaatgttaaattccaggaaagaaaaactatttacagtatatgctaggaatatttggaaacaatactaggaaatatgaatgtgcatgattaataagtattttttaaagttttcaaagagtatcagtaatcatacatctgtaatcttactgagaagtgagtctgtcttgttgctttctgaaatctttactgtgcattttcagttgtggattccactagggctgtatatacgcatctgctagtgatataccctttggatggtcaataaaaatgccaagtgaaaaacatttaaatcttctttttatttagcagttttcttccagaggtagcctcaggagaaatgatactggctgctctcttgtactttactaataatagtaatttaaagatgaagtatttgaaaagattggcatgtaagtcaggaagggacagttgcacagtttagattgaagagaaaataagtatctgtttgcttgttgccagattatccatcagcttaatgcaactgcaatttctcacttcgtatgacagtgtgtttataacaagaatttataattttgccatttcacttctcagtttgtgtgaccttatgtctcttgccatagctacttcttagagtgctgtgatatcggacacctttgacatctggtgggatttcctctgaatgcctaaggagaaactcatacaatttgtgtagagccatcccagcaggtacctttcaggcttgggagcttggaaaaatgctgatagaacacagtgtagaggaataaatgccaagagaatattcttgctacgggtagctgtggaaaatggacaacctacaggatagagtagtttcttagtaattctctggaaaggtaggggatgacttttccagctgtagtttcttggaccaaagcccaagcttcctatggatgtatcatagcaagaattcctggcaacataacagtgtctccaattctgccagcacaagcttgcttactgagttatctgtaaataacatgacacaaaggcatttccaaagtcaagactgtttttaggtaagatttagtgtatatttttattcactggaaaacgaaatgctatttattatagtccctcttagagtaccatgaagaatggatataacaaatgccaaagataagagttaatttatttataatatgtttaacaaatatttcaacatcaaagaaagtaaattttagtttttcaaataaagaaatatcttaatttctgttcatagacattaagcaaatattgaattgtttcaaaatgttatccctttagatagaataaaggttttcttgtttgtatatttttgttttgaattctttaggtattaaaagtgtgtagaggctaatgttagtcaaagtgtctgtgtttagaactccctcccacaaactagatattttataagttttgtttacctcccttaactagagtttgagaggtaggtggttgctggctcaaagatttcagagtttagttcttcaaattttttttaccctattctttgtggccttcttatggttacaagataggtgctccatctctaacattatatccatatttcaggcagaaaaaaggagagaaaaaaagcagaaaggctaaaaagaaaaaaataacaaggctaaaaaagcaaaaaatagcaacaaggctaacaaagaaaaaaaaggaggaaaataaagctgagtttgctccgtttttgagtaattgctcaatccaattaaatgtcattggccagaattgtattgtatggcctctcctctctgccagacagctgattattgttttttacatgataacatgatgatctcccagcccctaaaatgacattctcttatgaaagaagacagaaagggaaggaaatcagtctatcacaaaaatccatctttattgctacctcttaaataattttcaaatctattcatatttctgtatttccatttatatcatgttttaacagacaaggaataagaaatcagttaattgaattgatcagggagggtctcagggaggagatgagacttgaaaatgggttttgaggtttagctattgcttggagaagagaggaaggtaggaattccaagcaaaagggaagaaaggataaaagctccaagatggacgtgatcatggtacatacatatgagtgtgattatggttatgggcaaagagacaattaggagataagactttcttgatctgagatgtttgagacaatcttttttttttatactttaagtttta

SEQ ID NO: 9318 - RNA, 4704 nt, Homo sapiens
  source 1..4704: mol_type = other RNA
agctacagttacttttgcaccaacctaatatttcacagccactctcctggatgtttctggggagcttcagtctaggctcagacatggtgcctgctggttctgggaaaaggttaaggggctgagtagtagcacacactacatcctccagactgtctatgccatggctatgtttggaaaccctgcaaatggcctggcagagtctcaccttgccaatccagagaggatgtgggggatttctggcttaagaataggctgaaaagagggactggaggttactgccacatagccaagcattcctgggaactttctgggaatgtgaactgatatgaaaatggcttagactacaagaattatagggaaatatcagaatacccacctaaaaatggcttaaataagaaggccattttaaagcttacttcatgaggaattttgaaataggcagttccagggtcagtttggctgctcaacagagtcttcaaggacggaggcactcttcataattctcttctgccatcatcaggattcagtgaaatctccctctatggtcacaggatgactccagcagttctgattatcctgggttcagcaataactgcgttggttctcgtttcctcagtctttccctcttcttggaggatgagagccagaagtcacccaacttgtactggtatctgaactatataggtgaggaaggataaaaattcgaatctagggatttatgtaaatcttgactcttctactccaggacactgaagattatgtttacatttgtttgactgactgttgtctcaggttgctgtgtctcctggggatggctctgtgtggtccacccaaagctgaacagctgctttagatctttattgttgtcgtagcagtggagactgtgtaggttggtagcctcagagcaacaggctataccatccagcctaggcgtatagtaggctattccatctcaatttgtgtaagtacattccatgatgttcataaaacaacaaaatcacccacaatgcatttctcagaatgtatccttattgttaagtgacaaatgactgtatatagttttaactaaataaagttacctggagctcagtccctgagaacatgtctcctgtttaaacaagaatagaaagatgttaaaggcctactagtactaaactgaaatttttctccttgatactaggaaattaaaaggggaaacactttgtctctacctgatttagagtgtttaatgtaccattaccacctaaaatgatgtcccagattactagttgaagcattccatacattgggaaatactagattaaagaaacaaagagaaaggatcaaatagcctcactcactctcccattcattcatttctcttgttatgggcctgaaactgggtatgtagtgttgaacaacaaaaaccaaattcctgcccccattgacttaaccattgaacacggatcttttcttccttgtaacctattctatcatgcatctactcttgctctgtcaaattcttttcatcccagctcttatctcattgctgtcccaatatagtgtaactcatttggaggactagaaattccttgaagttcttgttctcctctgacatcagaccagtccctatgtgtaaggccaagccttggaatgtgcctggaaggctctgtctctggttcacaggctagatctccaagcctctagcaaatttggacaatacgtcatatctctcatgtctttcctgaaattcctgcatgatcagagaagttggggaggcaggggggtatatctaataataagaggtccaggatcatgattattctttcttttgtgctactatttagtgacaagttaggttttaatccaaaagtgtgctctggggcctcaagtacaaaatcaggctgcctcaattgtcttaacattgcctggtagaatcccttaaatgaggggtggttaatgcaaaatatatgtattttattaatatattatttggtatattagtaagtgcttttttaggtttccatataaaatctttcctccaatgttattaccaagcctcagaacttcttcagagttaatgcctgtgaactcctcatttaatgccccattgttctcacagaaattaattacagcgaatgttgtctgacttcatgggagtttaatgacagagattatgacctcacattccctttgcagaaggaaagcaggtgtggccaagaccggctttactaaaagcctcccactacatctttattcgaagaaatatagttatctatagttagaacttggaacttccaaattgtatttgttgttctgactgaacttttgtcaaattatataagtgcttcgataaggagttgtatctctcccattacccttctaaatttagaaatgataatttttgacatcctctaggggaagaaaattcttgaaagctctgataaaagcaaatttgttaacaaatttaaaaggtaatgttaatgttaaattccaggaaagaaaaactatttacagtatatgctaggaatatttggaaacaatactaggaaatatgaatgtgcatgattaataagtattttttaaagttttcaaagagtatcagtaatcatacatctgtaatcttactgagaagtgagtctgtcttgttgctttctgaaatctttactgtgcattttcagttgtggattccactagggctgtatatacgcatctgctagtgatataccctttggatggtcaataaaaatgccaagtgaaaaacatttaaatcttctttttatttagcagttttcttccagaggtagcctcaggagaaatgatactggctgctctcttgtactttactaataatagtaatttaaagatgaagtatttgaaaagattggcatgtaagtcaggaagggacagttgcacagtttagattgaagagaaaataagtatctgtttgcttgttgccagattatccatcagcttaatgcaactgcaatttctcacttcgtatgacagtgtgtttataacaagaatttataattttgccatttcacttctcagtttgtgtgaccttatgtctcttgccatagctacttcttagagtgctgtgatatcggacacctttgacatctggtgggatttcctctgaatgcctaaggagaaactcatacaatttgtgtagagccatcccagcaggtacctttcaggcttgggagcttggaaaaatgctgatagaacacagtgtagaggaataaatgccaagagaatattcttgctacgggtagctgtggaaaatggacaacctacaggatagagtagtttcttagtaattctctggaaaggtaggggatgacttttccagctgtagtttcttggaccaaagcccaagcttcctatggatgtatcatagcaagaattcctggcaacataacagtgtctccaattctgccagcacaagcttgcttactgagttatctgtaaataacatgacacaaaggcatttccaaagtcaagactgtttttaggtaagatttagtgtatatttttattcactggaaaacgaaatgctatttattatagtccctcttagagtaccatgaagaatggatataacaaatgccaaagataagagttaatttatttataatatgtttaacaaatatttcaacatcaaagaaagtaaattttagtttttcaaataaagaaatatcttaatttctgttcatagacattaagcaaatattgaattgtttcaaaatgttatccctttagatagaataaaggttttcttgtttgtatatttttgttttgaattctttaggtattaaaagtgtgtagaggctaatgttagtcaaagtgtctgtgtttagaactccctcccacaaactagatattttataagttttgtttacctcccttaactagagtttgagaggtaggtggttgctggctcaaagatttcagagtttagttcttcaaattttttttaccctattctttgtggccttcttatggttacaagataggtgctccatctctaacattatatccatatttcaggcagaaaaaaggagagaaaaaaagcagaaaggctaaaaagaaaaaaataacaaggctaaaaaagcaaaaaatagcaacaaggctaacaaagaaaaaaaaggaggaaaataaagctgagtttgctccgtttttgagtaattgctcaatccaattaaatgtcattggccagaattgtattgtatggcctctcctctctgccagacagctgattattgttttttacatgataacatgatgatctcccagcccctaaaatgacattctcttatgaaagaagacagaaagggaaggaaatcagtctatcacaaaaatccatctttattgctacctcttaaataattttcaaatctattcatatttctgtatttccatttatatcatgttttaacagacaaggaataagaaatcagttaattgaattgatcagggagggtctcagggaggagatgagacttgaaaatgggttttgaggtttagctattgcttggagaagagaggaaggtaggaattccaagcaaaagggaagaaaggataaaagctccaagatggacgtgatcatggtacatacatatgagtgtgattatggttatgggcaaagagacaattaggagataagactttcttgatctgagatgtttgagacaatcttttttttttatactttaagtttta

SEQ ID NO: 9319 - RNA, 1529 nt, Homo sapiens
  source 1..1529: mol_type = other RNA
agctacagttacttttgcaccaacctaatatttcacagccactctcctggatgtttctggggagcttcagtctaggctcagacatggtgcctgctggttctgggaaaaggttaaggggctgagtagtagcacacactacatcctccagactgtctatgccatggctatgtttggaaaccctgcaaatggcctggcagagtctcaccttgccaatccagagaggatgtgggggatttctggcttaagaataggctgaaaagagggactggaggttactgccacatagccaagcattcctgggaactttctgggaatgtgaactgatatgaaaatggcttagactacaagaattatagggaaatatcagaatacccacctaaaaatggcttaaataagaaggccattttaaagcttacttcatgaggaattttgaaataggcagttccagggtcagtttggctgctcaacagagtcttcaaggacggaggcactcttcataattctcttctgccatcatcaggattcagtgaaatctccctctatggtcacaggatgactccagcagttctgattatcctgggttcagcaataactgcgttggttctcgtttcctcagtctttccctcttcttggaggatgagagccagaagtcacccaacttgtactggtatctgaactatataggtgaggaaggataaaaattcgaatctagggatttatgtaaatcttgactcttctactctttatgccaggctctgttctcaggactactcatgaaataactcacagaatccatacagcaaccttatgaaggaggtctgaggggagtccccattttacatgtgaattacgctgtgaggcaagggagctgaagtagtttgccaaaggtcacacacctagtaagtaggggaacagattcaaacaagaatgagacagacattttctgttatttttcacatgcaaaaatgtctctattctacctcaccatttgattaataattctgggctaagaaataatttcttttagaatttgaaggcttgttcttataacttttaacttgtaatatttttttgagaaatctaagccattttgatttctcattctttgcatatggctagtttttggttcttgggtttagtatcttttcattatctctgattttgaaattttatgataatgagcattaataattaatacgggttttgaaaaaaatgtgctggacagttgatgggccattttatatgatacatggtcttcattttggggaaggtttattttcgtcctcttttgatcccatcattatccctctgatttctctttggagcatgcatttattcattcaacaaatagttatcatgcccctcccctagcaaggcattgtaattctgtgctagaggtaatagcagtgaacaaaacattgccctcatggagccaatttgatattgggccttcttgattgaccctttaattagcttgtttttcctgtagtccatcctttcaactactttatattattttctgaaatatt

SEQ ID NO: 9320 - RNA, 7147 nt, Homo sapiens
  source 1..7147: mol_type = other RNA
agctacagttacttttgcaccaacctgataactcttcaaaatgtttggtgaggctggactcaaacataagtgcatggatgcctgatttttttcccccagtattcaagaacctcagggttttcctgaatgtgctatagacattccagggacctcctaagttttgaacattgcattattatgaagattaggtccataagttttatcagattttctaaaatacgagtaaacattttttaaacccaaggtttgctgccaacttctctcctctacagatcctggaaagaagaaagaaatggcttctaacaaaaagaaggggaggatttccagctcatttctaattcaggctcattggagaaggaagtggcatgggtgacgataagcagcagtttttatgtctgaaggaaactgaaaacagcatctcactggggtggccaggagctcttctgctgaagtctctgtgtatccagaatgcctgggattggattcttgtcctgttgcctctgacttcctagaagtggcctctgggccgtctttatttattaaatcatctgggtatgatctggctctgatattttggcattcgggagtggcagaccaagctcaaattgcaatagtcctttaaaaagatgtttctaaaagccagatatgcactgacatttcagaaagaacatttgtgcctaatttccagctgccaagttatagttcatcattcagcttcatattggaggccttcaggctttgatttatttaggaaacattggtgaacaatgggatcatgatctgcaacatgacagatgtaggaagtccatgtcccctaaaggaggttttctggagactcctaacaattaagagaatctgttctgtttctaagttgacagcaaattattgaattctgagtatccagaatgagtttggggagtaagagttgtgaagggcagacattaactgcttatttaagacataatacctgtcctttggaaacttatggtttgttagggggtagtgtcctagaaacaatgtaagacaatttgttaccaaatgataaatagaactttaaaacaaaaattttcctactgtcagggaaactaagttttccttttctttgaaggcatggagaagtgccgagcagtgtgttacttttcctctattccctggttcgttcctcacccacgtcagtttttcttcatatttgtctttattggaacccacaaagtttattcaaagttattatcagtttcttcccttttgtgaagaaaattcaatttttatgaattagatttttaagatggcttgtaatgtacccatacagccaggtataagaaattacctggtagcttcactgatgcagatgacagatacctgtggggacttacagtctagttgggagagtaatcacacacatacacacacacacacacacacacaccccagatttggcatgagaagaacaacgctgaagtcgatatctgcctattttgtttataatggtgtgaccttgggcaagtcacttaatttttcaatgtattttctcatctataagatgggagatatcttatatcctaaggctattgattatgtcagatggaatctcatctgagaaaataccttagaaattgtacagtatgataaaaatattgacttttattttctaaatcatacatagcaagatgcaggactagtttaattgttgtcacttttagaatccgattttcacatcatcattccatttcttatgatatttaacatgacaagcaaaagaccttgttcaaaggggaagaacaaataagattaattctctgtaaatcctttaaaattttattatccatctcttcactggggaaatgtctagatacattttcctaagtggttccatctttctgtaaatggctattgacctgctgagtgcagttttgctttcagagaagcattgcacttggtgtgtgatttgagtttgggatcatgaccttatttcctttgcacttgattgctttacttcaccaactgcatccctgattttgatattatctgtggctagctcctttcatgattttgggaatggctacctctcagttttctgaatattttttagtacttgctgttacaatgtagacattgcaataatgttctaaaattatatgtacatttacttactcaacacaaatttaaagagtacctgataagagctggtactctgagtactgagcactgagtacctggtagaatcattaatacagaagacaaagctctggcctcaaggattctgcagtacagcagcagggaggtaaaacacacataccacatttgtttactgcaagtgtgggaggtagataggtgtcccctaaaaacatgtgttcccagaacctgtgacgtgaccttacttggaaaaagggtctttgcagatgtttaagttaataatcttgtgatgagatcatcctggattgtacaggtgggccctaaatccagtgaaaactatctttgtaagagacagatgaggagaagacgtagagacttgtgaaacagaaggccatgtgaagacagaggcagagattggagggatataaccagaaagaatgcccataggcagcagaaattggaagaggtaagaattggattgttgcctaaagccttcagaaggagtgtgaccctgtcagcatttggatctccgactctggcctttaaaactgagagagaaaaaaatttctgttgttttaagccagtgagtttgtggtaattttttaatggcagccatgagaaacgaatacaacaaggaacaggataatctacaaaatacatgaattatacaagagcatcagaagtttgtggaaatttagtataaaaaacacctcttattgaaagtgtgattgttactatacagtcagtccagaagcactgaattatgaaaatatcattgcctggtatgtgtcagttatgtttataataatataaataatctaagcacacattgtgtcctgtaattttaattttactctaacatcccatgcaaaggtttaactgtaggtggccatttcatgaaacaaatgccaatttctcatggaccaatgttctcccagcagaggaaatatatcttcctgcccacactgggctacaacatcactaaaattacaagcagaaaggaggtctgcatttctatagcctcttcttttcttatctagtagtaaatggttataaacttgacattttccagttacaaacataagtaataatattgtaataacaaaagggaaggtccaatcctatagatcccactgatggtgatagagtaaatcaaggaatttggaagaagtggtatctagtttcacaagttgaaaaaccagaattatcttcaggcattcataatttcagtgtcatgggttaaggtgtttgggggcaaaatgagtttctggctgtgggatggatttgagtggtgttagcaatcattcaataacagaagccactgaagcagccttcgtctccctaatcaaaatgctgccatcataccattttgctcccaaaatatgctaaaagtaaggcaccaacggtaataagtagtataggtaatttttaagtaccataaaagtttacaatattaacagttacatttgttaattttgtctggcttagttggtggtgacttcagatggtaactgggtggaataagacttctaagcccacataagacaggatggtgtgatctttctgggagggtgccacgtctgtccaatattgatacaatagtgcaccagtggcagcttcttggttgggccaagtaagccttctcaatgtatttactccttcagtatttataacaatcaggaagctgtaattattgtccatattttactaatgaagtaactaaaacttagagaagataagcaatttgtctgaggtcatgctctagtagtgagcagagccagaatctgaactctggcatgatgactatagcgtctgtgtttttatgcattactgataggtatgggtggtatactggagacttagtgagtatttaggtgtgagtaacgtctacagtgacgtcagggagctcactgtacatccatgacatgagaaataaaattcccacgcttccctgtcttgaagctgaggcaatatattacatgggttaactgacaattcagacagagtgagagattcattatattcaccacaaatgaacacagatggacactcttcaaataaagcttcctattgaattttaatagtgctcttctgcagaacacatttgaaaaatggatcatagcatattcatattttcctttagcttgccaaatgtgagatgattaagaaacctgcttaaactttaaatattcttaccatacacatgcatttttcaaatgtatgcgtctgcaataaatatttgttaaatgaatatgaatgtatatacacaaacatacatgaagcaataggcgcacacacatttaatttgataaatatttgttgagtatctactgaatataaacttgggctgaagagttatggaaatacaaagacagaattcttttctgttcccaagaagctttataaggggaagtgagacatgctcagtcttgttctggtggcagctctcaaagtgtggtctctggctcggcagtgttggcatcacttggggacttgttagaaatggaaatgcttgtgccccaccatacacctgctaaatgagaaactgtggctgggggtctagcaatttatggttgtaaaagtcctccagggaactctgatgcacgttaaaatttcagaaccactgggcacaggaacgctttaatgtgctaaaggatgctaaatattactttcacgtggagacatctgagaaggcttgaagaaagagattgtatttgagcagagtcttggagaacaggtagattttggctgatagaaacagagaagggaaataaagtcaaagagaagagaggaagtcaacttagctcgtttgagttggcagataggctgcccatggatgaaaacccagattaaaatcaggcagtggaaatccctgagcaacacgcttgtgagtttagacattgttctgaaagacattggcagtcattgaaggtttctgagtggggaagaagtgtgatcaaaactaccttccttttttttttttcttacccagtgaatgtaattcagcacttgtactgagttcatattaacagaacttgatggttgtaaatcagtcttttcttcctcattaaaatcacttcaccattaagaattatctataggttatggctggaatcatgttatctctgctctttcttgactattctgacacagcaggcaacttaatttcaacaactcggtaatgcccccatcttctgtgtgtgtgtgtgtgtgtgtgtgtgtgtgtgtgtgtggtgtttgctaagaaggagtcacacggctgcttttgaattcagctgggctttaggaagctgcataaaaacaaagaaaaaatgttgctgcttgctagtgcattctttgttatgtagcaatcagaaggatgactgtgctctgaagtggtgcaggtggcctcttctgatactaattccagcgtctcaactagttcagcatcaaaagggagttctctggaagggaaataattctgtccctacccctgattgctcctatttgcccagcattgtgggcacctgcttggccacccaccttccttttctttgccatccacttgcgtcatctttctcttcccctgggtcagcctgtatatttcaatctatccacaccctgcgcaagctcattcattcatgggctttctctctgcaattttcattgtgcctccctttgttggcataattgattccctgctttgcaagagcaggtggatgagttggtttattcctttaaaaaattcctcctcttttctctttcattgctctgatctttagtcaatctttggttcagccagcttgttctccttctattgactaatctctctctgtatctttcataatggtggtgggagagtccatgccgaatctccctaattataagtattgtgttgctaaaaattgctgatgataatctgagcatacagtgggtcataatcttcttacttgtgaagggtcttgccttgatattgacggctgctcactgatcagggtagtggttgctgaaggaggttagggtggctgtagcaatttcctaaaataagacaacaatgaagtttgctttatcaattaactcttgcttttatgaaagatatctttgtagcatacgatgctgtttgatagcattttacccacagtagaacttctttcaaaattagaatgaattcactcaaaacttgcaggtgctttatcaactgaatttatggaatattctaaatcctttgtagtcatttcaacaatgttcacagcatctttaccaggagaaaattccattttaagaaactactttctttgctcatctatagaagcaactcttaaaatccattccagttttatcatgagatggcagcaattcagtcacagcttcagtttctacctctagttctagttctcttgctacttccaccacatctgcatctactttctccactgatgttttgaacccttcagccatccatgaagattggaatcttttccaaactcctgttaatgttgatatttcaaacttctcccatgaatcacgaatgttctttatggcatttacaatgttaaatcattttcaaaaaattttccatttgctttatccatatctatcagaggaatcaccatgtcagttctagccttacaaagtgtattttttaaataataagacttgaaagttgaaattattccttgattcatgggctagagaatggatgttacgttagcagacatgaaagccacattaatcttcttgtactcccatcaaagttctggagtgactaggtgcattgtcaatgaatagtaacattttgaaaaaaaaaaaaatcttttttttttccttagcagtagttctcaatagtaggcttaaagtattcagtaaaccattttgtaaatagatgtactgtcatccaggctttgttgttccatttacagagcacaggcagagtagattttgctaaattctggggccctaggattttttgaatggtatataagcattggcttcaacttaaagtcaccagctgccttagcccccaacaatatagtca

SEQ ID NO: 9321 - RNA, 28 nt, Homo sapiens
  source 1..28: mol_type = other RNA
agctacagttacttttgcaccaatctaa

SEQ ID NO: 9322 - RNA, 1038 nt, Homo sapiens
  source 1..1038: mol_type = other RNA
agctacattgtctgctgggtttctccactataaaggtactatatttcccaggattaaacagatacgaacaatccaccatcatgtgaattggctctctgattattgcaaaacaagattcattaaaatggatgatcttctggacacagtcaaatgatggaagagaataatcataacgtaacatgaaaaataatagcatgtatcaaatagtggttaccccaaggcagagaggacctctaacatttcatgcagtgttatcaggtttacagatgattcttgaatgtttttctttttctttttaacacttctatcaggcagaggaaaatggtcttctagaaactcgcccaaggtactcaagagtttctccttatattcttttatattaagcattttagttttcagttcattaaagattcttgattcagaaaatgtttcaaccttatttttcaattcactgtgtagtacattaagagattccattatctgttgctgttcatccaaccaccgttgttccctttctaagtcttcctttaacttttcattctttgactccttagtggacagtaccatttcaagatcttgtctcagcttttggaactcttcttttcctaatgttatgagaacgtcttcagtcaagggaattgtttcaggtgtttttttctgccattgactgagttcagcggttaaacattttacttgcataattaacaatgatagctgagcatttgaatcggtgagtgtttcagttccaataagtgataatttattctgacattcttccatatctttccacatttcttcacattctctaataagttcttcttcagtatttgtaacatctcccacatctgtagtactatccggatctagatcctcctggaagagggtcatcaacagaaccagaaaatgatggcacccagatcttgaatctccagcctctagaccatcacagcgtcacaaactccaggtcgcctaggcgctgcgcaggaagcgcttgccagccccggacttctgcgcgcgctgcatgcccattggatgtgc

SEQ ID NO: 9323 - RNA, 855 nt, Homo sapiens
  source 1..855: mol_type = other RNA
agctacattgtctgctgggtttctccactataaaggtactatatttccctctaacatttcatgcagtgttatcaggtttacagatgattcttgaatgtttttctttttctttttaacacttctatcaggcagaggaaaatggtcttctagaaactcgcccaaggtactcaagagtttctccttatattcttttatattaagcattttagttttcagttcattaaagattcttgattcagaaaatgtttcaaccttatttttcaattcactgtgtagtacattaagagattccattatctgttgctgttcatccaaccaccgttgttccctttctaagtcttcctttaacttttcattctttgactccttagtggacagtaccatttcaagatcttgtctcagcttttggaactcttcttttcctaatgttatgagaacgtcttcagtcaagggaattgtttcaggtgtttttttctgccattgactgagttcagcggttaaacattttacttgcataattaacaatgatagctgagcatttgaatcggtgagtgtttcagttccaataagtgataatttattctgacattcttccatatctttccacatttcttcacattctctaataagttcttcttcagtatttgtaacatctcccacatctgtagtactatccggatctagatcctcctggaagagggtcatcaacagaaccagaaaatgatggcacccagatcttgaatctccagcctctagaccatcacagcgtcacaaactccaggtcgcctaggcgctgcgcaggaagcgcttgccagccccggacttctgcgcgcgctgcatgcccattggatgtgc

SEQ ID NO: 9324 - RNA, 79 nt, Homo sapiens
  source 1..79: mol_type = other RNA
agctcatccatagttgtcactgatttgagacagtgacaactatggatgagctctcaatatattcttgagttgcatgtct

SEQ ID NO: 9325 - RNA, 1507 nt, Homo sapiens
  source 1..1507: mol_type = other RNA
agctccctgaatccctgtcccagcaggtgcatcccggccccacgccccaggcacccctgcaggccgagtccgcccggaactcaagaccaagcagcagatcctgaagcagcggcgccgggcccagaagctgcacttcctgcagcgtggtggcctcaagcagctctctgcccgcaaccgccgccgcgtccaggagctgcagcagggcgccttcggccggggtgcccgctccaagaagggcaagatgcggaagaggatgtgaggaccaggacccagccccgtggctccttgattggccttagggtgggcatcagcagacgttcccgtgcaccactgtgtgcctggccctgtgctgggcactgggggcactccctgcaggagccatcatctgtgaaaaggagcactgtatggccacagaagggcagcagctgcgtcagcctgtgtcagggctaggaggcaggggctgcaggctcagcctgacccaggccggccagcatggcagagaggtcctgcatgaacagcttcacgtgctctagctgtccctccgtgtcctcgatgtccagggtgggaggctgcccctgatgctggcacactagctggaacaggttgagcacagccatcctgctgcgtcccaggagcagagtcttctccgctgctgtgttctgaatctgaatccacttggattcccactgcagcgtacgctccctggcagcctccaggcgctcctgcagctgtgcccgccgctggccctgtgcgagcacctcgtccggccaggcgtcccgcagctgctgcagccgcgctcgcgccgcctccagctccgcgagctgctcgcgctccctgagcctcagcgccgcctgcgtctcggccaggccgtcgaagcgcgccaccagctccggaacctcttggaacccgggcagcagctccagcgcttgctccagcaggcgcgcgcagggctccaggcgcttaagccggcgctgcagccgcgcgtgttcccgccgtagctcctggagctgggtccacagacgcagcgcctccacctcccgacggcccgcctggtgcctctcctccgccgccctccgcagcgcgcgattgcgccgggcctcggagtcctgcaaaaacttgtcaaagcggatgaacgatccctttagctcccgctccttttgttccagctgttcccaacgctgtttcagggctgccgtcttggtgcggaacacctccttctgggcctgcagggcctggtctgcatctaccagctcttgcctcttctccaggagacgcagtactggtgggacatgatcctcagcctgctctggcagctttgtagacagtttctcttgcaaagccagtcggaaatattcctcccagggcaccgccatccttctggcagttgccccagctttctttccaccagctggagttttgcacaagcttaggagaccctgggggttctgtggagcgtggtgtggaagcctgctcagctcggcccagaaggcagccaccagcaggctct

SEQ ID NO: 9326 - RNA, 30 nt, Homo sapiens
  source 1..30: mol_type = other RNA
agctcggtctgaggcccctcagtcttgctt

SEQ ID NO: 9327 - RNA, 2455 nt, Homo sapiens
  source 1..2455: mol_type = other RNA
agctggtaaaatggaaccaaatgatcatctaaagtttaaaattcctaaattgtccaatttatacaactgtgggagacttattcaaggtttttgaaagtccaggactgtttcagctgaaccagagggcacacaatttgcatcactgaaactgtcctgggttagtcaatgaaataaaaatgtctaaccacatacacatggatatgatctttgtcggttagattattgataaagtcagtctcagacaagtttccaaactgtgctatttaactagatacaattgagaaattctcaaatgaaaattttatatagtgtcatatcaatcaaaagaaaataatgaaactaagaatacagatcactgttggaagagaaagcagtggtgatggtgtgggtactgcaggaggtggtggggccgtggcacactagaaaagttgggtcacgctgagtaggaagcatttgattttctctggtgcttttagctctggggccggtcaaaggcctctctctggcatggctgtccagggtttgtcccaatgtgtctgagtgagccagcttgagaaggggtcgtgccgtttcttctttcacacaggggaaaaaaaagaccaaacacggaggtgcccagggtgtggatctgctggtgtcccgggagaaccagctggctgggcagcccttcttccccacaggcagctgctattgcgtagggaccgccaggtcaccgagtggccatcacaacaaaccccagcacagtccagcccggccacagccgcctccttgtgtttctgttgtcttccctgctgctgcccacatcctttacccaccgtgtctctcggcccactggaggtatcagaaattccaaattttcaaagcagtttcagtattttcagtatatatgttgggattttataatggttcatggccagaaaaggttcagcacctcccacacacagacattggtccgtttcctgttcttggcatctctgtactttgttggtccaactcagacagcaactttaagatgttcagcgcagccatatcatggcaggactccacatccttgccgataccatggctgatcagaggtggctgagaggagcaattgataagagatacaaattcgttcttgttgtttttggggaagtctttgtattcaacctggaatccctggactctggaaagatagtccagttgctcagagggtctcgtgagaggtccatggggtacgtggcctgaagagatgttattctttaaaatggtctcggctgtgggcgaggtgcccccatacaacaactctcgggctatcatggcagttaccgtggccttggcaggattcggagctgccctggtaaaatctttggtgtgatgtccttgactaactcctacagcctgggcgacctcgggcaccatgggaagaattccagcaggcagctgctgatgacttagataaggcatcctgaactcatcctctttattactagtcccattttcatccccagagccaggttcaaaaaaggttacttttcttccatcccctggtttctttatgggtgtcttctcctctgacttgagtgcgggtttggtgggctgcgcctgcgggactttgaaaccaaggatctccagcatgttctcggctgcattgcgcttggccaccttcttgttggtgcccgttccttctgcagtgtggtttccaaccttcacctgcatcacaaactccctgcggcgcgggaggcctcgctctgtgaggagcgtgtactctggctccttctccttttttgcctgctggatctgggccagtcggctaatcggattgatcccctggccatattctgggcttgtctgtggcttgactatgggttttgttttctttttgattctaggctttactcgttcaactgcaggcaggggcggtaacttcttcagctcctcaagaacagctatggcggcatttttctttgaaatcttcttgcttttcccttcaccttcccccacaaactccccaaccgaaaccttggtcacaaagttcttcatgtggggtgggccactctcccgggccacctcgaaattcacaggcaagttccgtttaagtgcaatctcaaacacttgacttatttcagatttattgagattttcttcttcggattctcttccattcacctccagcctctctggcaggggctcattctgcaggatcctcaacgctttggcagcagcatcgtgtttcgcagcctgtcttgtctttcctttgccattaaattgctgtcctcccacagaaagttccacttgataaagtaaaggtggaactggaaatgggtaaaagtacctcgggggataagcacctcctctcatgttgtagttataggtggactgcatccgagagtaagggtcaacaggcttatacattggtttttttccaagtttcatgcacagtgcatttagttctacagtaggggttatgctttct

SEQ ID NO: 9328 - RNA, 2961 nt, Homo sapiens
  source 1..2961: mol_type = other RNA
agctggtaaaatggaaccaaatgatcatctaaagtttaaaattcctaaattgtccaatttatacaactgtgggagacttattcaaggtttttgaaagtccaggactgtttcagctgaaccagagggcacacaatttgcatcactgaaactgtcctgggttagtcaatgaaataaaaatgtctaaccacatacacatggatatgatctttgtcggttagattattgataaagtcagtctcagacaagtttccaaactgtgctatttaactagatacaattgagaaattctcaaatgaaaattttatatagtgtcatatcaatcaaaagaaaataatgaaactaagaatacagatcactgttggaagagaaagcagtggtgatggtgtgggtactgcaggaggtggtggggccgtggcacactagaaaagttgggtcacgctgagtaggaagcatttgattttctctggtgcttttagctctggggccggtcaaaggcctctctctggcatggctgtccagggtttgtcccaatgtgtctgagtgagccagcttgagaaggggtcgtgccgtttcttctttcacacaggggaaaaaaaagaccaaacacggaggtgcccagggtgtggatctgctggtgtcccgggagaaccagctggctgggcagcccttcttccccacaggcagctgctattgcgtagggaccgccaggtcaccgagtggccatcacaacaaaccccagcacagtccagcccggccacagccgcctccttgtgtttctgttgtcttccctgctgctgcccacatcctttacccaccgtgtctctcggcccactggaggtatcagaaattccaaattttcaaagcagtttcagtattttcagtatatatgttgggattttataatggttcatggccagaaaaggttcagcacctcccacacacagacattggtccgtttcctgttcttggcatctctgtactttgttggtccaactcagacagcaactttaagatgttcagcgcagccatatcatggcaggactccacatccttgccgataccatggctgatcagaggtggctgagaggagcaattgataagagatacaaattcgttcttgttgtttttggggaagtctttgtattcaacctggaatccctggactctggaaagatagtccagttgctcagagggtctcgtgagaggtccatggggtacgtggcctgaagagatgttattctttaaaatggtctcggctgtgggcgaggtgcccccatacaacaactctcgggctatcatggcagttaccgtggccttggcaggattcggagctgccctggtaaaatctttggtgtgatgtccttgactaactcctacagcctgggcgacctcgggcaccatgggaagaattccagcaggcagctgctgatgacttagataaggcatcctgaactcatcctctttattactagtcccattttcatccccagagccaggttcaaaaaaggttacttttcttccatcccctggtttctttatgggtgtcttctcctctgacttgagtgcgggtttggtgggctgcgcctgcgggactttgaaaccaaggatctccagcatgttctcggctgcattgcgcttggccaccttcttgttggtgcccgttccttctgcagtgtggtttccaaccttcacctgcatcacaaactccctgcggcgcgggaggcctcgctctgtgaggagcgtgtactctggctccttctccttttttgcctgctggatctgggccagtcggctaatcggattgatcccctggccatattctgggcttgtctgtggcttgactatgggttttgttttctttttgattctaggctttactcgttcaactgcaggcaggggcggtaacttcttcagctcctcaagaacagctatggcggcatttttctttgaaatcttcttgcttttcccttcaccttcccccacaaactccccaaccgaaaccttggtcacaaagttcttcatgtggggtgggccactctcccgggccacctcgaaattcacaggcaagttccgtttaagtgcaatctcaaacacttgacttatttcagatttattgagattttcttcttcggattctcttccattcacctccagcctctctggcaggggctcattctgcaggatcctcaacgctttggcagcagcatcgtgtttcgcagcctgtcttgtctttcctttgccattaaattgctgtcctcccacagaaagttccacttgataaagtaaaggtggaactggaaatgggtaaaagtacctcgggggataagcacctcctctcatgttgtagttataggtggactgcatccgagagtaagggtcaacaggcttatacattggtttttttccaagtttcatgcacagtgcatttagttctacagtaggggttatgctttctgcagctgcactggtggatgtaatagatgcagagggtaaagcagagttttgaatgggtctacctgcattttcagagggcagagagctagtagtagaaggaatactcatcaaaggctgtgagagaagagactggttcttgttcagtatttggctccctgagagagcagcagatgggttctgaacttgcacttgaacttgagacatggtcactttcaacaaaagtgaacaaatgcaggtaaacagctttcagtgcaggttaattcagtgctatgaagtctaaagttctacctggctgctgctccgagctcgtcccccggccggcggtcctgggcggtggcggcgaggaggggaaggaagaaggaaaaaagggagaggaagaagggacgaagggagggaagaggcggagtggccgtggaggaggcgggcgccgccgggccgggggggggaggcggtcaaaggaagcgggagccgagagagacgcggcagccgccggcgcaaacgctgaag

SEQ ID NO: 9329 - RNA, 3036 nt, Homo sapiens
  source 1..3036: mol_type = other RNA
agctggtaaaatggaaccaaatgatcatctaaagtttaaaattcctaaattgtccaatttatacaactgtgggagacttattcaaggtttttgaaagtccaggactgtttcagctgaaccagagggcacacaatttgcatcactgaaactgtcctgggttagtcaatgaaataaaaatgtctaaccacatacacatggatatgatctttgtcggttagattattgataaagtcagtctcagacaagtttccaaactgtgctatttaactagatacaattgagaaattctcaaatgaaaattttatatagtgtcatatcaatcaaaagaaaataatgaaactaagaatacagatcactgttggaagagaaagcagtggtgatggtgtgggtactgcaggaggtggtggggccgtggcacactagaaaagttgggtcacgctgagtaggaagcatttgattttctctggtgcttttagctctggggccggtcaaaggcctctctctggcatggctgtccagggtttgtcccaatgtgtctgagtgagccagcttgagaaggggtcgtgccgtttcttctttcacacaggggaaaaaaaagaccaaacacggaggtgcccagggtgtggatctgctggtgtcccgggagaaccagctggctgggcagcccttcttccccacaggcagctgctattgcgtagggaccgccaggtcaccgagtggccatcacaacaaaccccagcacagtccagcccggccacagccgcctccttgtgtttctgttgtcttccctgctgctgcccacatcctttacccaccgtgtctctcggcccactggaggtatcagaaattccaaattttcaaagcagtttcagtattttcagtatatatgttgggattttataatggttcatggccagaaaaggttcagcacctcccacacacagacattggtccgtttcctgttcttggcatctctgtactttgttggtccaactcagacagcaactttaagatgttcagcgcagccatatcatggcaggactccacatccttgccgataccatggctgatcagaggtggctgagaggagcaattgataagagatacaaattcgttcttgttgtttttggggaagtctttgtattcaacctggaatccctggactctggaaagatagtccagttgctcagagggtctcgtgagaggtccatggggtacgtggcctgaagagatgttattctttaaaatggtctcggctgtgggcgaggtgcccccatacaacaactctcgggctatcatggcagttaccgtggccttggcaggattcggagctgccctggtaaaatctttggtgtgatgtccttgactaactcctacagcctgggcgacctcgggcaccatgggaagaattccagcaggcagctgctgatgacttagataaggcatcctgaactcatcctctttattactagtcccattttcatccccagagccaggttcaaaaaaggttacttttcttccatcccctggtttctttatgggtgtcttctcctctgacttgagtgcgggtttggtgggctgcgcctgcgggactttgaaaccaaggatctccagcatgttctcggctgcattgcgcttggccaccttcttgttggtgcccgttccttctgcagtgtggtttccaaccttcacctgcatcacaaactccctgcggcgcgggaggcctcgctctgtgaggagcgtgtactctggctccttctccttttttgcctgctggatctgggccagtcggctaatcggattgatcccctggccatattctgggcttgtctgtggcttgactatgggttttgttttctttttgattctaggctttactcgttcaactgcaggcaggggcggtaacttcttcagctcctcaagaacagctatggcggcatttttctttgaaatcttcttgcttttcccttcaccttcccccacaaactccccaaccgaaaccttggtcacaaagttcttcatgtggggtgggccactctcccgggccacctcgaaattcacaggcaagttccgtttaagtgcaatctcaaacacttgacttatttcagatttattgagattttcttcttcggattctcttccattcacctccagcctctctggcaggggctcattctgcaggatcctcaacgctttggcagcagcatcgtgtttcgcagcctgtcttgtctttcctttgccattaaattgctgtcctcccacagaaagttccacttgataaagtaaaggtggaactggaaatgggtaaaagtacctcgggggataagcacctcctctcatgttgtagttataggtggactgcatccgagagtaagggtcaacaggcttatacattggtttttttccaagtttcatgcacagtgcatttagttctacagtaggggttatgctttctgcagctgcactggtggatgtaatagatgcagagggtaaagcagagttttgaatgggtctacctgcattttcagagggcagagagctagtagtagaaggaatactcatcaaaggctgtgagagaagagactggttcttgttcagtatttggctccctgagagagcagcagatgggttctgaacttgcacttgaacttgagacatggtcactttcaacaaaagtgaacaaatgcaggtaaacagctttcagtgcaggttaattcagtgctatgaagtctaaagttctaccttttttaaaaagagggcgttccaggaacaatgttgtctttgttcagttctgagaggttaagtggttaataaactctggctgctgctccgagctcgtcccccggccggcggtcctgggcggtggcggcgaggaggggaaggaagaaggaaaaaagggagaggaagaagggacgaagggagggaagaggcggagtggccgtggaggaggcgggcgccgccgggccgggggggggaggcggtcaaaggaagcgggagccgagagagacgcggcagccgccggcgcaaacgctgaag

SEQ ID NO: 9330 - RNA, 3159 nt, Homo sapiens
  source 1..3159: mol_type = other RNA
agctggtaaaatggaaccaaatgatcatctaaagtttaaaattcctaaattgtccaatttatacaactgtgggagacttattcaaggtttttgaaagtccaggactgtttcagctgaaccagagggcacacaatttgcatcactgaaactgtcctgggttagtcaatgaaataaaaatgtctaaccacatacacatggatatgatctttgtcggttagattattgataaagtcagtctcagacaagtttccaaactgtgctatttaactagatacaattgagaaattctcaaatgaaaattttatatagtgtcatatcaatcaaaagaaaataatgaaactaagaatacagatcactgttggaagagaaagcagtggtgatggtgtgggtactgcaggaggtggtggggccgtggcacactagaaaagttgggtcacgctgagtaggaagcatttgattttctctggtgcttttagctctggggccggtcaaaggcctctctctggcatggctgtccagggtttgtcccaatgtgtctgagtgagccagcttgagaaggggtcgtgccgtttcttctttcacacaggggaaaaaaaagaccaaacacggaggtgcccagggtgtggatctgctggtgtcccgggagaaccagctggctgggcagcccttcttccccacaggcagctgctattgcgtagggaccgccaggtcaccgagtggccatcacaacaaaccccagcacagtccagcccggccacagccgcctccttgtgtttctgttgtcttccctgctgctgcccacatcctttacccaccgtgtctctcggcccactggaggtatcagaaattccaaattttcaaagcagtttcagtattttcagtatatatgttgggattttataatggttcatggccagaaaaggttcagcacctcccacacacagacattggtccgtttcctgttcttggcatctctgtactttgttggtccaactcagacagcaactttaagatgttcagcgcagccatatcatggcaggactccacatccttgccgataccatggctgatcagaggtggctgagaggagcaattgataagagatacaaattcgttcttgttgtttttggggaagtctttgtattcaacctggaatccctggactctggaaagatagtccagttgctcagagggtctcgtgagaggtccatggggtacgtggcctgaagagatgttattctttaaaatggtctcggctgtgggcgaggtgcccccatacaacaactctcgggctatcatggcagttaccgtggccttggcaggattcggagctgccctggtaaaatctttggtgtgatgtccttgactaactcctacagcctgggcgacctcgggcaccatgggaagaattccagcaggcagctgctgatgacttagataaggcatcctgaactcatcctctttattactagtcccattttcatccccagagccaggttcaaaaaaggttacttttcttccatcccctggtttctttatgggtgtcttctcctctgacttgagtgcgggtttggtgggctgcgcctgcgggactttgaaaccaaggatctccagcatgttctcggctgcattgcgcttggccaccttcttgttggtgcccgttccttctgcagtgtggtttccaaccttcacctgcatcacaaactccctgcggcgcgggaggcctcgctctgtgaggagcgtgtactctggctccttctccttttttgcctgctggatctgggccagtcggctaatcggattgatcccctggccatattctgggcttgtctgtggcttgactatgggttttgttttctttttgattctaggctttactcgttcaactgcaggcaggggcggtaacttcttcagctcctcaagaacagctatggcggcatttttctttgaaatcttcttgcttttcccttcaccttcccccacaaactccccaaccgaaaccttggtcacaaagttcttcatgtggggtgggccactctcccgggccacctcgaaattcacaggcaagttccgtttaagtgcaatctcaaacacttgacttatttcagatttattgagattttcttcttcggattctcttccattcacctccagcctctctggcaggggctcattctgcaggatcctcaacgctttggcagcagcatcgtgtttcgcagcctgtcttgtctttcctttgccattaaattgctgtcctcccacagaaagttccacttgataaagtaaaggtggaactggaaatgggtaaaagtacctcgggggataagcacctcctctcatgttgtagttataggtggactgcatccgagagtaagggtcaacaggcttatacattggtttttttccaagtttcatgcacagtgcatttagttctacagtaggggttatgctttctgcagctgcactggtggatgtaatagatgcagagggtaaagcagagttttgaatgggtctacctgcattttcagagggcagagagctagtagtagaaggaatactcatcaaaggctgtgagagaagagactggttcttgttcagtatttggctccctgagagagcagcagatgggttctgaacttgcacttgaacttgagacatggtcactttcaacaaaagtgaacaaatgcaggtaaacagctttcagtgcaggttaattcagtgctatgaagtctaaagttctaccttttttaaaaagagggcgttccaggaacaatgttgtctttgttcagttctgagaggttaagtggttaataaactctgtaatctcagcttatcgggaggctgaagtgggaaaatcgcttgaacctgggaggtggaggttgcagtgagccgagatcacgccactgcactccagcctgggcgacaagagcaaaactccacctggctgctgctccgagctcgtcccccggccggcggtcctgggcggtggcggcgaggaggggaaggaagaaggaaaaaagggagaggaagaagggacgaagggagggaagaggcggagtggccgtggaggaggcgggcgccgccgggccgggggggggaggcggtcaaaggaagcgggagccgagagagacgcggcagccgccggcgcaaacgctgaag

SEQ ID NO: 9331 - RNA, 2983 nt, Homo sapiens
  source 1..2983: mol_type = other RNA
agctggtaaaatggaaccaaatgatcatctaaagtttaaaattcctaaattgtccaatttatacaactgtgggagacttattcaaggtttttgaaagtccaggactgtttcagctgaaccagagggcacacaatttgcatcactgaaactgtcctgggttagtcaatgaaataaaaatgtctaaccacatacacatggatatgatctttgtcggttagattattgataaagtcagtctcagacaagtttccaaactgtgctatttaactagatacaattgagaaattctcaaatgaaaattttatatagtgtcatatcaatcaaaagaaaataatgaaactaagaatacagatcactgttggaagagaaagcagtggtgatggtgtgggtactgcaggaggtggtggggccgtggcacactagaaaagttgggtcacgctgagtaggaagcatttgattttctctggtgcttttagctctggggccggtcaaaggcctctctctggcatggctgtccagggtttgtcccaatgtgtctgagtgagccagcttgagaaggggtcgtgccgtttcttctttcacacaggggaaaaaaaagaccaaacacggaggtgcccagggtgtggatctgctggtgtcccgggagaaccagctggctgggcagcccttcttccccacaggcagctgctattgcgtagggaccgccaggtcaccgagtggccatcacaacaaaccccagcacagtccagcccggccacagccgcctccttgtgtttctgttgtcttccctgctgctgcccacatcctttacccaccgtgtctctcggcccactggaggtatcagaaattccaaattttcaaagcagtttcagtattttcagtatatatgttgggattttataatggttcatggccagaaaaggttcagcacctcccacacacagacattggtccgtttcctgttcttggcatctctgtactttgttggtccaactcagacagcaactttaagatgttcagcgcagccatatcatggcaggactccacatccttgccgataccatggctgatcagaggtggctgagaggagcaattgataagagatacaaattcgttcttgttgtttttggggaagtctttgtattcaacctggaatccctggactctggaaagatagtccagttgctcagagggtctcgtgagaggtccatggggtacgtggcctgaagagatgttattctttaaaatggtctcggctgtgggcgaggtgcccccatacaacaactctcgggctatcatggcagttaccgtggccttggcaggattcggagctgccctggtaaaatctttggtgtgatgtccttgactaactcctacagcctgggcgacctcgggcaccatgggaagaattccagcaggcagctgctgatgacttagataaggcatcctgaactcatcctctttattactagtcccattttcatccccagagccaggttcaaaaaaggttacttttcttccatcccctggtttctttatgggtgtcttctcctctgacttgagtgcgggtttggtgggctgcgcctgcgggactttgaaaccaaggatctccagcatgttctcggctgcattgcgcttggccaccttcttgttggtgcccgttccttctgcagtgtggtttccaaccttcacctgcatcacaaactccctgcggcgcgggaggcctcgctctgtgaggagcgtgtactctggctccttctccttttttgcctgctggatctgggccagtcggctaatcggattgatcccctggccatattctgggcttgtctgtggcttgactatgggttttgttttctttttgattctaggctttactcgttcaactgcaggcaggggcggtaacttcttcagctcctcaagaacagctatggcggcatttttctttgaaatcttcttgcttttcccttcaccttcccccacaaactccccaaccgaaaccttggtcacaaagttcttcatgtggggtgggccactctcccgggccacctcgaaattcacaggcaagttccgtttaagtgcaatctcaaacacttgacttatttcagatttattgagattttcttcttcggattctcttccattcacctccagcctctctggcaggggctcattctgcaggatcctcaacgctttggcagcagcatcgtgtttcgcagcctgtcttgtctttcctttgccattaaattgctgtcctcccacagaaagttccacttgataaagtaaaggtggaactggaaatgggtaaaagtacctcgggggataagcacctcctctcatgttgtagttataggtggactgcatccgagagtaagggtcaacaggcttatacattggtttttttccaagtttcatgcacagtgcatttagttctacagtaggggttatgctttctgcagctgcactggtggatgtaatagatgcagagggtaaagcagagttttgaatgggtctacctgcattttcagagggcagagagctagtagtagaaggaatactcatcaaaggctgtgagagaagagactggttcttgttcagtatttggctccctgagagagcagcagatgggttctgaacttgcacttgaacttgagacatggtcactttcaacaaaagtgaacaaatgcaggtaaacagctttcagtgcaggttaattcagtgctatgaagtctaaagttctaccttttttaaaaagagggcgttccaggaacaatgttgtctttgttcagttctgagaggttaagtggttaataaactcttctttcctcctccacttcctttttccttccttgctgtcgcttcttcctcttgtcctgcctctggccttcctttctctccttcctgcagttgtttcttcctccatctaaaaagctccgccccttgatggcgtcacacgaaaccaaccacgccccatattgccgca

SEQ ID NO: 9332 - RNA, 2672 nt, Homo sapiens
  source 1..2672: mol_type = other RNA
agctggtaaaatggaaccaaatgatcatctaaagtttaaaattcctaaattgtccaatttatacaactgtgggagacttattcaaggtttttgaaagtccaggactgtttcagctgaaccagagggcacacaatttgcatcactgaaactgtcctgggttagtcaatgaaataaaaatgtctaaccacatacacatggatatgatctttgtcggttagattattgataaagtcagtctcagacaagtttccaaactgtgctatttaactagatacaattgagaaattctcaaatgaaaattttatatagtgtcatatcaatcaaaagaaaataatgaaactaagaatacagatcactgttggaagagaaagcagtggtgatggtgtgggtactgcaggaggtggtggggccgtggcacactagaaaagttgggtcacgctgagtaggaagcatttgattttctctggtgcttttagctctggggccggtcaaaggcctctctctggcatggctgtccagggtttgtcccaatgtgtctgagtgagccagcttgagaaggggtcgtgccgtttcttctttcacacaggggaaaaaaaagaccaaacacggaggtgcccagggtgtggatctgctggtgtcccgggagaaccagctggctgggcagcccttcttccccacaggcagctgctattgcgtagggaccgccaggtcaccgagtggccatcacaacaaaccccagcacagtccagcccggccacagccgcctccttgtgtttctgttgtcttccctgctgctgcccacatcctttacccaccgtgtctctcggcccactggaggtatcagaaattccaaattttcaaagcagtttcagtattttcagtatatatgttgggattttataatggttcatggccagaaaaggttcagcacctcccacacacagacattggtccgtttcctgttcttggcatctctgtactttgttggtccaactcagacagcaactttaagatgttcagcgcagccatatcatggcaggactccacatccttgccgataccatggctgatcagaggtggctgagaggagcaattgataagagatacaaattcgttcttgttgtttttggggaagtctttgtattcaacctggaatccctggactctggaaagatagtccagttgctcagagggtctcgtgagaggtccatggggtacgtggcctgaagagatgttattctttaaaatggtctcggctgtgggcgaggtgcccccatacaacaactctcgggctatcatggcagttaccgtggccttggcaggattcggagctgccctggtaaaatctttggtgtgatgtccttgactaactcctacagcctgggcgacctcgggcaccatgggaagaattccagcaggcagctgctgatgacttagataaggcatcctgaactcatcctctttattactagtcccattttcatccccagagccaggttcaaaaaaggttacttttcttccatcccctggtttctttatgggtgtcttctcctctgacttgagtgcgggtttggtgggctgcgcctgcgggactttgaaaccaaggatctccagcatgttctcggctgcattgcgcttggccaccttcttgttggtgcccgttccttctgcagtgtggtttccaaccttcacctgcatcacaaactccctgcggcgcgggaggcctcgctctgtgaggagcgtgtactctggctccttctccttttttgcctgctggatctgggccagtcggctaatcggattgatcccctggccatattctgggcttgtctgtggcttgactatgggttttgttttctttttgattctaggctttactcgttcaactgcaggcaggggcggtaacttcttcagctcctcaagaacagctatggcggcatttttctttgaaatcttcttgcttttcccttcaccttcccccacaaactccccaaccgaaaccttggtcacaaagttcttcatgtggggtgggccactctcccgggccacctcgaaattcacaggcaagttccgtttaagtgcaatctcaaacacttgacttatttcagatttattgagattttcttcttcggattctcttccattcacctccagcctctctggcaggggctcattctgcaggatcctcaacgctttggcagcagcatcgtgtttcgcagcctgtcttgtctttcctttgccattaaattgctgtcctcccacagaaagttccacttgataaagtaaaggtggaactggaaatgggtaaaagtacctcgggggataagcacctcctctcatgttgtagttataggtggactgcatccgagagtaagggtcaacaggcttatacattggtttttttccaagtttcatgcacagtgcatttagttctacagtaggggttatgctttctggctgctgctccgagctcgtcccccggccggcggtcctgggcggtggcggcgaggaggggaaggaagaaggaaaaaagggagaggaagaagggacgaagggagggaagaggcggagtggccgtggaggaggcgggcgccgccgggccgggggggggaggcggtcaaaggaagcgggagccgagagagacgcggcagccgccggcgcaaacgctgaag

SEQ ID NO: 9333 - RNA, 3049 nt, Homo sapiens
  source 1..3049: mol_type = other RNA
agctggtaaaatggaaccaaatgatcatctaaagtttaaaattcctaaattgtccaatttatacaactgtgggagacttattcaaggtttttgaaagtccaggactgtttcagctgaaccagagggcacacaatttgcatcactgaaactgtcctgggttagtcaatgaaataaaaatgtctaaccacatacacatggatatgatctttgtcggttagattattgataaagtcagtctcagacaagtttccaaactgtgctatttaactagatacaattgagaaattctcaaatgaaaattttatatagtgtcatatcaatcaaaagaaaataatgaaactaagaatacagatcactgttggaagagaaagcagtggtgatggtgtgggtactgcaggaggtggtggggccgtggcacactagaaaagttgggtcacgctgagtaggaagcatttgattttctctggtgcttttagctctggggccggtcaaaggcctctctctggcatggctgtccagggtttgtcccaatgtgtctgagtgagccagcttgagaaggggtcgtgccgtttcttctttcacacaggggaaaaaaaagaccaaacacggaggtgcccagggtgtggatctgctggtgtcccgggagaaccagctggctgggcagcccttcttccccacaggcagctgctattgcgtagggaccgccaggtcaccgagtggccatcacaacaaaccccagcacagtccagcccggccacagccgcctccttgtgtttctgttgtcttccctgctgctgcccacatcctttacccaccgtgtctctcggcccactggaggtatcagaaattccaaattttcaaagcagtttcagtattttcagtatatatgttgggattttataatggttcatggccagaaaaggttcagcacctcccacacacagacattggtccgtttcctgttcttggcatctctgtactttgttggtccaactcagacagcaactttaagatgttcagcgcagccatatcatggcaggactccacatccttgccgataccatggctgatcagaggtggctgagaggagcaattgataagagatacaaattcgttcttgttgtttttggggaagtctttgtattcaacctggaatccctggactctggaaagatagtccagttgctcagagggtctcgtgagaggtccatggggtacgtggcctgaagagatgttattctttaaaatggtctcggctgtgggcgaggtgcccccatacaacaactctcgggctatcatggcagttaccgtggccttggcaggattcggagctgccctggtaaaatctttggtgtgatgtccttgactaactcctacagcctgggcgacctcgggcaccatgggaagaattccagcaggcagctgctgatgacttagataaggcatcctgaactcatcctctttattactagtcccattttcatccccagagccaggttcaaaaaaggttacttttcttccatcccctggtttctttatgggtgtcttctcctctgacttgagtgcgggtttggtgggctgcgcctgcgggactttgaaaccaaggatctccagcatgttctcggctgcattgcgcttggccaccttcttgttggtgcccgttccttctgcagtgtggtttccaaccttcacctgcatcacaaactccctgcggcgcgggaggcctcgctctgtgaggagcgtgtactctggctccttctccttttttgcctgctggatctgggccagtcggctaatcggattgatcccctggccatattctgggcttgtctgtggcttgactatgggttttgttttctttttgattctaggctttactcgttcaactgcaggcaggggcggtaacttcttcagctcctcaagaacagctatggcggcatttttctttgaaatcttcttgcttttcccttcaccttcccccacaaactccccaaccgaaaccttggtcacaaagttcttcatgtggggtgggccactctcccgggccacctcgaaattcacaggcaagttccgtttaagtgcaatctcaaacacttgacttatttcagatttattgagattttcttcttcggattctcttccattcacctccagcctctctggcaggggctcattctgcaggatcctcaacgctttggcagcagcatcgtgtttcgcagcctgtcttgtctttcctttgccattaaattgctgtcctcccacagaaagttccacttgataaagtaaaggtggaactggaaatgggtaaaagtacctcgggggataagcacctcctctcatgttgtagttataggtggactgcatccgagagtaagggtcaacaggcttatacattggtttttttccaagtttcatgcacagtgcatttagttctacagtaggggttatgctttcttcatagctgatttttcttgtaggtcttacttttaggattccctcagtgcacggcttccacccccttgacacttcacacatcaggacatcaggggtctcctttattatatgttctgcagtccatcaggctactcatttaagtacaaacaacagcatgaactcaaaaccctggcaggcaggaaggtcaaatggcagaagcctgcaacgcagtacaatccctgggtcatcttggtgattgtctcatggataaatgctgaaggggaaaaagcttttttaaaaagagggcgttccaggaacaatgttgtctttgttcagttctgagaggttaagtggttaataaactctggctgctgctccgagctcgtcccccggccggcggtcctgggcggtggcggcgaggaggggaaggaagaaggaaaaaagggagaggaagaagggacgaagggagggaagaggcggagtggccgtggaggaggcgggcgccgccgggccgggggggggaggcggtcaaaggaagcgggagccgagagagacgcggcagccgccggcgcaaacgctgaagagccgctcaggcgcccgcagcccggcaggaagt

SEQ ID NO: 9334 - RNA, 3139 nt, Homo sapiens
  source 1..3139: mol_type = other RNA
agctggtaaaatggaaccaaatgatcatctaaagtttaaaattcctaaattgtccaatttatacaactgtgggagacttattcaaggtttttgaaagtccaggactgtttcagctgaaccagagggcacacaatttgcatcactgaaactgtcctgggttagtcaatgaaataaaaatgtctaaccacatacacatggatatgatctttgtcggttagattattgataaagtcagtctcagacaagtttccaaactgtgctatttaactagatacaattgagaaattctcaaatgaaaattttatatagtgtcatatcaatcaaaagaaaataatgaaactaagaatacagatcactgttggaagagaaagcagtggtgatggtgtgggtactgcaggaggtggtggggccgtggcacactagaaaagttgggtcacgctgagtaggaagcatttgattttctctggtgcttttagctctggggccggtcaaaggcctctctctggcatggctgtccagggtttgtcccaatgtgtctgagtgagccagcttgagaaggggtcgtgccgtttcttctttcacacaggggaaaaaaaagaccaaacacggaggtgcccagggtgtggatctgctggtgtcccgggagaaccagctggctgggcagcccttcttccccacaggcagctgctattgcgtagggaccgccaggtcaccgagtggccatcacaacaaaccccagcacagtccagcccggccacagccgcctccttgtgtttctgttgtcttccctgctgctgcccacatcctttacccaccgtgtctctcggcccactggaggtatcagaaattccaaattttcaaagcagtttcagtattttcagtatatatgttgggattttataatggttcatggccagaaaaggttcagcacctcccacacacagacattggtccgtttcctgttcttggcatctctgtactttgttggtccaactcagacagcaactttaagatgttcagcgcagccatatcatggcaggactccacatccttgccgataccatggctgatcagaggtggctgagaggagcaattgataagagatacaaattcgttcttgttgtttttggggaagtctttgtattcaacctggaatccctggactctggaaagatagtccagttgctcagagggtctcgtgagaggtccatggggtacgtggcctgaagagatgttattctttaaaatggtctcggctgtgggcgaggtgcccccatacaacaactctcgggctatcatggcagttaccgtggccttggcaggattcggagctgccctggtaaaatctttggtgtgatgtccttgactaactcctacagcctgggcgacctcgggcaccatgggaagaattccagcaggcagctgctgatgacttagataaggcatcctgaactcatcctctttattactagtcccattttcatccccagagccaggttcaaaaaaggttacttttcttccatcccctggtttctttatgggtgtcttctcctctgacttgagtgcgggtttggtgggctgcgcctgcgggactttgaaaccaaggatctccagcatgttctcggctgcattgcgcttggccaccttcttgttggtgcccgttccttctgcagtgtggtttccaaccttcacctgcatcacaaactccctgcggcgcgggaggcctcgctctgtgaggagcgtgtactctggctccttctccttttttgcctgctggatctgggccagtcggctaatcggattgatcccctggccatattctgggcttgtctgtggcttgactatgggttttgttttctttttgattctaggctttactcgttcaactgcaggcaggggcggtaacttcttcagctcctcaagaacagctatggcggcatttttctttgaaatcttcttgcttttcccttcaccttcccccacaaactccccaaccgaaaccttggtcacaaagttcttcatgtggggtgggccactctcccgggccacctcgaaattcacaggcaagttccgtttaagtgcaatctcaaacacttgacttatttcagatttattgagattttcttcttcggattctcttccattcacctccagcctctctggcaggggctcattctgcaggatcctcaacgctttggcagcagcatcgtgtttcgcagcctgtcttgtctttcctttgccattaaattgctgtcctcccacagaaagttccacttgataaagtaaaggtggaactggaaatgggtaaaagtacctcgggggataagcacctcctctcatgttgtagttataggtggactgcatccgagagtaagggtcaacaggcttatacattggtttttttccaagtttcatgcacagtgcatttagttctacagtaggggttatgctttcttcatagctgatttttcttgtaggtcttacttttaggattccctcagtgcacggcttccacccccttgacacttcacacatcaggacatcaggggtctcctttattatatgttctgcagtccatcaggctactcatttaagtacaaacaacagcatgaactcaaaaccctggcaggcaggaaggtcaaatggcagaagcctgcaacgcagtacaatccctgggtcatcttggtgattgtctcatggataaatgctgaaggggaaaaagcttttttaaaaagagggcgttccaggaacaatgttgtctttgttcagttctgagaggttaagtggttaataaactctgtaatctcagcttatcgggaggctgaagtgggaaaatcgcttgaacctgggaggtggaggttgcagtgagccgagatcacgccactgcactccagcctgggcgacaagagcaaaactccacctggctgctgctccgagctcgtcccccggccggcggtcctgggcggtggcggcgaggaggggaaggaagaaggaaaaaagggagaggaagaagggacgaagggagggaagaggcggagtggccgtggaggaggcgggcgccgccgggccgggggggggaggcggtcaaaggaagcgggagccgagagagacgcggcagccgccggcgcaaacgctgaag

SEQ ID NO: 9335 - RNA, 2747 nt, Homo sapiens
  source 1..2747: mol_type = other RNA
agctggtaaaatggaaccaaatgatcatctaaagtttaaaattcctaaattgtccaatttatacaactgtgggagacttattcaaggtttttgaaagtccaggactgtttcagctgaaccagagggcacacaatttgcatcactgaaactgtcctgggttagtcaatgaaataaaaatgtctaaccacatacacatggatatgatctttgtcggttagattattgataaagtcagtctcagacaagtttccaaactgtgctatttaactagatacaattgagaaattctcaaatgaaaattttatatagtgtcatatcaatcaaaagaaaataatgaaactaagaatacagatcactgttggaagagaaagcagtggtgatggtgtgggtactgcaggaggtggtggggccgtggcacactagaaaagttgggtcacgctgagtaggaagcatttgattttctctggtgcttttagctctggggccggtcaaaggcctctctctggcatggctgtccagggtttgtcccaatgtgtctgagtgagccagcttgagaaggggtcgtgccgtttcttctttcacacaggggaaaaaaaagaccaaacacggaggtgcccagggtgtggatctgctggtgtcccgggagaaccagctggctgggcagcccttcttccccacaggcagctgctattgcgtagggaccgccaggtcaccgagtggccatcacaacaaaccccagcacagtccagcccggccacagccgcctccttgtgtttctgttgtcttccctgctgctgcccacatcctttacccaccgtgtctctcggcccactggaggtatcagaaattccaaattttcaaagcagtttcagtattttcagtatatatgttgggattttataatggttcatggccagaaaaggttcagcacctcccacacacagacattggtccgtttcctgttcttggcatctctgtactttgttggtccaactcagacagcaactttaagatgttcagcgcagccatatcatggcaggactccacatccttgccgataccatggctgatcagaggtggctgagaggagcaattgataagagatacaaattcgttcttgttgtttttggggaagtctttgtattcaacctggaatccctggactctggaaagatagtccagttgctcagagggtctcgtgagaggtccatggggtacgtggcctgaagagatgttattctttaaaatggtctcggctgtgggcgaggtgcccccatacaacaactctcgggctatcatggcagttaccgtggccttggcaggattcggagctgccctggtaaaatctttggtgtgatgtccttgactaactcctacagcctgggcgacctcgggcaccatgggaagaattccagcaggcagctgctgatgacttagataaggcatcctgaactcatcctctttattactagtcccattttcatccccagagccaggttcaaaaaaggttacttttcttccatcccctggtttctttatgggtgtcttctcctctgacttgagtgcgggtttggtgggctgcgcctgcgggactttgaaaccaaggatctccagcatgttctcggctgcattgcgcttggccaccttcttgttggtgcccgttccttctgcagtgtggtttccaaccttcacctgcatcacaaactccctgcggcgcgggaggcctcgctctgtgaggagcgtgtactctggctccttctccttttttgcctgctggatctgggccagtcggctaatcggattgatcccctggccatattctgggcttgtctgtggcttgactatgggttttgttttctttttgattctaggctttactcgttcaactgcaggcaggggcggtaacttcttcagctcctcaagaacagctatggcggcatttttctttgaaatcttcttgcttttcccttcaccttcccccacaaactccccaaccgaaaccttggtcacaaagttcttcatgtggggtgggccactctcccgggccacctcgaaattcacaggcaagttccgtttaagtgcaatctcaaacacttgacttatttcagatttattgagattttcttcttcggattctcttccattcacctccagcctctctggcaggggctcattctgcaggatcctcaacgctttggcagcagcatcgtgtttcgcagcctgtcttgtctttcctttgccattaaattgctgtcctcccacagaaagttccacttgataaagtaaaggtggaactggaaatgggtaaaagtacctcgggggataagcacctcctctcatgttgtagttataggtggactgcatccgagagtaagggtcaacaggcttatacattggtttttttccaagtttcatgcacagtgcatttagttctacagtaggggttatgctttcttttttaaaaagagggcgttccaggaacaatgttgtctttgttcagttctgagaggttaagtggttaataaactctggctgctgctccgagctcgtcccccggccggcggtcctgggcggtggcggcgaggaggggaaggaagaaggaaaaaagggagaggaagaagggacgaagggagggaagaggcggagtggccgtggaggaggcgggcgccgccgggccgggggggggaggcggtcaaaggaagcgggagccgagagagacgcggcagccgccggcgcaaacgctgaag

SEQ ID NO: 9336 - RNA, 2870 nt, Homo sapiens
  source 1..2870: mol_type = other RNA
agctggtaaaatggaaccaaatgatcatctaaagtttaaaattcctaaattgtccaatttatacaactgtgggagacttattcaaggtttttgaaagtccaggactgtttcagctgaaccagagggcacacaatttgcatcactgaaactgtcctgggttagtcaatgaaataaaaatgtctaaccacatacacatggatatgatctttgtcggttagattattgataaagtcagtctcagacaagtttccaaactgtgctatttaactagatacaattgagaaattctcaaatgaaaattttatatagtgtcatatcaatcaaaagaaaataatgaaactaagaatacagatcactgttggaagagaaagcagtggtgatggtgtgggtactgcaggaggtggtggggccgtggcacactagaaaagttgggtcacgctgagtaggaagcatttgattttctctggtgcttttagctctggggccggtcaaaggcctctctctggcatggctgtccagggtttgtcccaatgtgtctgagtgagccagcttgagaaggggtcgtgccgtttcttctttcacacaggggaaaaaaaagaccaaacacggaggtgcccagggtgtggatctgctggtgtcccgggagaaccagctggctgggcagcccttcttccccacaggcagctgctattgcgtagggaccgccaggtcaccgagtggccatcacaacaaaccccagcacagtccagcccggccacagccgcctccttgtgtttctgttgtcttccctgctgctgcccacatcctttacccaccgtgtctctcggcccactggaggtatcagaaattccaaattttcaaagcagtttcagtattttcagtatatatgttgggattttataatggttcatggccagaaaaggttcagcacctcccacacacagacattggtccgtttcctgttcttggcatctctgtactttgttggtccaactcagacagcaactttaagatgttcagcgcagccatatcatggcaggactccacatccttgccgataccatggctgatcagaggtggctgagaggagcaattgataagagatacaaattcgttcttgttgtttttggggaagtctttgtattcaacctggaatccctggactctggaaagatagtccagttgctcagagggtctcgtgagaggtccatggggtacgtggcctgaagagatgttattctttaaaatggtctcggctgtgggcgaggtgcccccatacaacaactctcgggctatcatggcagttaccgtggccttggcaggattcggagctgccctggtaaaatctttggtgtgatgtccttgactaactcctacagcctgggcgacctcgggcaccatgggaagaattccagcaggcagctgctgatgacttagataaggcatcctgaactcatcctctttattactagtcccattttcatccccagagccaggttcaaaaaaggttacttttcttccatcccctggtttctttatgggtgtcttctcctctgacttgagtgcgggtttggtgggctgcgcctgcgggactttgaaaccaaggatctccagcatgttctcggctgcattgcgcttggccaccttcttgttggtgcccgttccttctgcagtgtggtttccaaccttcacctgcatcacaaactccctgcggcgcgggaggcctcgctctgtgaggagcgtgtactctggctccttctccttttttgcctgctggatctgggccagtcggctaatcggattgatcccctggccatattctgggcttgtctgtggcttgactatgggttttgttttctttttgattctaggctttactcgttcaactgcaggcaggggcggtaacttcttcagctcctcaagaacagctatggcggcatttttctttgaaatcttcttgcttttcccttcaccttcccccacaaactccccaaccgaaaccttggtcacaaagttcttcatgtggggtgggccactctcccgggccacctcgaaattcacaggcaagttccgtttaagtgcaatctcaaacacttgacttatttcagatttattgagattttcttcttcggattctcttccattcacctccagcctctctggcaggggctcattctgcaggatcctcaacgctttggcagcagcatcgtgtttcgcagcctgtcttgtctttcctttgccattaaattgctgtcctcccacagaaagttccacttgataaagtaaaggtggaactggaaatgggtaaaagtacctcgggggataagcacctcctctcatgttgtagttataggtggactgcatccgagagtaagggtcaacaggcttatacattggtttttttccaagtttcatgcacagtgcatttagttctacagtaggggttatgctttcttttttaaaaagagggcgttccaggaacaatgttgtctttgttcagttctgagaggttaagtggttaataaactctgtaatctcagcttatcgggaggctgaagtgggaaaatcgcttgaacctgggaggtggaggttgcagtgagccgagatcacgccactgcactccagcctgggcgacaagagcaaaactccacctggctgctgctccgagctcgtcccccggccggcggtcctgggcggtggcggcgaggaggggaaggaagaaggaaaaaagggagaggaagaagggacgaagggagggaagaggcggagtggccgtggaggaggcgggcgccgccgggccgggggggggaggcggtcaaaggaagcgggagccgagagagacgcggcagccgccggcgcaaacgctgaag

SEQ ID NO: 9337 - RNA, 2973 nt, Homo sapiens
  source 1..2973: mol_type = other RNA
agctggtaaaatggaaccaaatgatcatctaaagtttaaaattcctaaattgtccaatttatacaactgtgggagacttattcaaggtttttgaaagtccaggactgtttcagctgaaccagagggcacacaatttgcatcactgaaactgtcctgggttagtcaatgaaataaaaatgtctaaccacatacacatggatatgatctttgtcggttagattattgataaagtcagtctcagacaagtttccaaactgtgctatttaactagatacaattgagaaattctcaaatgaaaattttatatagtgtcatatcaatcaaaagaaaataatgaaactaagaatacagatcactgttggaagagaaagcagtggtgatggtgtgggtactgcaggaggtggtggggccgtggcacactagaaaagttgggtcacgctgagtaggaagcatttgattttctctggtgcttttagctctggggccggtcaaaggcctctctctggcatggctgtccagggtttgtcccaatgtgtctgagtgagccagcttgagaaggggtcgtgccgtttcttctttcacacaggggaaaaaaaagaccaaacacggaggtgcccagggtgtggatctgctggtgtcccgggagaaccagctggctgggcagcccttcttccccacaggcagctgctattgcgtagggaccgccaggtcaccgagtggccatcacaacaaaccccagcacagtccagcccggccacagccgcctccttgtgtttctgttgtcttccctgctgctgcccacatcctttacccaccgtgtctctcggcccactggaggtatcagaaattccaaattttcaaagcagtttcagtattttcagtatatatgttgggattttataatggttcatggccagaaaaggttcagcacctcccacacacagacattggtccgtttcctgttcttggcatctctgtactttgttggtccaactcagacagcaactttaagatgttcagcgcagccatatcatggcaggactccacatccttgccgataccatggctgatcagaggtggctgagaggagcaattgataagagatacaaattcgttcttgttgtttttggggaagtctttgtattcaacctggaatccctggactctggaaagatagtccagttgctcagagggtctcgtgagaggtccatggggtacgtggcctgaagagatgttattctttaaaatggtctcggctgtgggcgaggtgcccccatacaacaactctcgggctatcatggcagttaccgtggccttggcaggattcggagctgccctggtaaaatctttggtgtgatgtccttgactaactcctacagcctgggcgacctcgggcaccatgggaagaattccagcaggcagctgctgatgacttagataaggcatcctgaactcatcctctttattactagtcccattttcatccccagagccaggttcaaaaaaggttacttttcttccatcccctggtttctttatgggtgtcttctcctctgacttgagtgcgggtttggtgggctgcgcctgcgggactttgaaaccaaggatctccagcatgttctcggctgcattgcgcttggccaccttcttgttggtgcccgttccttctgcagtgtggtttccaaccttcacctgcatcacaaactccctgcggcgcgggaggcctcgctctgtgaggagcgtgtactctggctccttctccttttttgcctgctggatctgggccagtcggctaatcggattgatcccctggccatattctgggcttgtctgtggcttgactatgggttttgttttctttttgattctaggctttactcgttcaactgcaggcaggggcggtaacttcttcagctcctcaagaacagctatggcggcatttttctttgaaatcttcttgcttttcccttcaccttcccccacaaactccccaaccgaaaccttggtcacaaagttcttcatgtggggtgggccactctcccgggccacctgtttcagagggaaagactcgaaattcacaggcaagttccgtttaagtgcaatctcaaacacttgacttatttcagatttattgagattttcttcttcggattctcttccattcacctccagcctctctggcaggggctcattctgcaggatcctcaacgctttggcagcagcatcgtgtttcgcagcctgtcttgtctttcctttgccattaaattgctgtcctcccacagaaagttccacttgataaagtaaaggtggaactggaaatgggtaaaagtacctcgggggataagcacctcctctcatgttgtagttataggtggactgcatccgagagtaagggtcaacaggcttatacattggtttttttccaagtttcatgcacagtgcatttagttctacagtaggggttatgctttcccccttgacacttcacacatcaggacatcaggggtctcctttattatatgttctgcagtccatcaggctactcatttaagtacaaacaacagcatgaactcaaaaccctggcaggcaggaaggtcaaatggcagaagcctgcaacgcagtacaatccctgggtcatcttggtgattgtctcatggataaatgctgaaggggaaaaagcttttttaaaaagagggcgttccaggaacaatgttgtctttgttcagttctgagaggttaagtggttaataaactctggctgctgctccgagctcgtcccccggccggcggtcctgggcggtggcggcgaggaggggaaggaagaaggaaaaaagggagaggaagaagggacgaagggagggaagaggcggagtggccgtggaggaggcgggcgccgccgggccgggggggggaggcggtcaaaggaagcgggagccgagagagacgcggcagccgccggcgcaaacgctgaag

SEQ ID NO: 9338 - RNA, 2979 nt, Homo sapiens
  source 1..2979: mol_type = other RNA
agctggtaaaatggaaccaaatgatcatctaaagtttaaaattcctaaattgtccaatttatacaactgtgggagacttattcaaggtttttgaaagtccaggactgtttcagctgaaccagagggcacacaatttgcatcactgaaactgtcctgggttagtcaatgaaataaaaatgtctaaccacatacacatggatatgatctttgtcggttagattattgataaagtcagtctcagacaagtttccaaactgtgctatttaactagatacaattgagaaattctcaaatgaaaattttatatagtgtcatatcaatcaaaagaaaataatgaaactaagaatacagatcactgttggaagagaaagcagtggtgatggtgtgggtactgcaggaggtggtggggccgtggcacactagaaaagttgggtcacgctgagtaggaagcatttgattttctctggtgcttttagctctggggccggtcaaaggcctctctctggcatggctgtccagggtttgtcccaatgtgtctgagtgagccagcttgagaaggggtcgtgccgtttcttctttcacacaggggaaaaaaaagaccaaacacggaggtgcccagggtgtggatctgctggtgtcccgggagaaccagctggctgggcagcccttcttccccacaggcagctgctattgcgtagggaccgccaggtcaccgagtggccatcacaacaaaccccagcacagtccagcccggccacagccgcctccttgtgtttctgttgtcttccctgctgctgcccacatcctttacccaccgtgtctctcggcccactggaggtatcagaaattccaaattttcaaagcagtttcagtattttcagtatatatgttgggattttataatggttcatggccagaaaaggttcagcacctcccacacacagacattggtccgtttcctgttcttggcatctctgtactttgttggtccaactcagacagcaactttaagatgttcagcgcagccatatcatggcaggactccacatccttgccgataccatggctgatcagaggtggctgagaggagcaattgataagagatacaaattcgttcttgttgtttttggggaagtctttgtattcaacctggaatccctggactctggaaagatagtccagttgctcagagggtctcgtgagaggtccatggggtacgtggcctgaagagatgttattctttaaaatggtctcggctgtgggcgaggtgcccccatacaacaactctcgggctatcatggcagttaccgtggccttggcaggattcggagctgccctggtaaaatctttggtgtgatgtccttgactaactcctacagcctgggcgacctcgggcaccatgggaagaattccagcaggcagctgctgatgacttagataaggcatcctgaactcatcctctttattactagtcccattttcatccccagagccaggttcaaaaaaggttacttttcttccatcccctggtttctttatgggtgtcttctcctctgacttgagtgcgggtttggtgggctgcgcctgcgggactttgaaaccaaggatctccagcatgttctcggctgcattgcgcttggccaccttcttgttggtgcccgttccttctgcagtgtggtttccaaccttcacctgcatcacaaactccctgcggcgcgggaggcctcgctctgtgaggagcgtgtactctggctccttctccttttttgcctgctggatctgggccagtcggctaatcggattgatcccctggccatattctgggcttgtctgtggcttgactatgggttttgttttctttttgattctaggctttactcgttcaactgcaggcaggggcggtaacttcttcagctcctcaagaacagctatggcggcatttttctttgaaatcttcttgcttttcccttcaccttcccccacaaactccccaaccgaaaccttggtcacaaagttcttcatgtggggtgggccactctcccgggccacctgtttcagagggaaagactcgaaattcacaggcaagttccgtttaagtgcaatctcaaacacttgacttatttcagatttattgagattttcttcttcggattctcttccattcacctccagcctctctggcaggggctcattctgcaggatcctcaacgctttggcagcagcatcgtgtttcgcagcctgtcttgtctttcctttgccattaaattgctgtcctcccacagaaagttccacttgataaagtaaaggtggaactggaaatgggtaaaagtacctcgggggataagcacctcctctcatgttgtagttataggtggactgcatccgagagtaagggtcaacaggcttatacattggtttttttccaagtttcatgcacagtgcatttagttctacagtaggggttatgctttctgcagctgcactggtggatgtaatagatgcagagggtaaagcagagttttgaatgggtctacctgcattttcagagggcagagagctagtagtagaaggaatactcatcaaaggctgtgagagaagagactggttcttgttcagtatttggctccctgagagagcagcagatgggttctgaacttgcacttgaacttgagacatggtcactttcaacaaaagtgaacaaatgcaggtaaacagctttcagtgcaggttaattcagtgctatgaagtctaaagttctacctggctgctgctccgagctcgtcccccggccggcggtcctgggcggtggcggcgaggaggggaaggaagaaggaaaaaagggagaggaagaagggacgaagggagggaagaggcggagtggccgtggaggaggcgggcgccgccgggccgggggggggaggcggtcaaaggaagcgggagccgagagagacgcggcagccgccggcgcaaacgctgaag

SEQ ID NO: 9339 - RNA, 3054 nt, Homo sapiens
  source 1..3054: mol_type = other RNA
agctggtaaaatggaaccaaatgatcatctaaagtttaaaattcctaaattgtccaatttatacaactgtgggagacttattcaaggtttttgaaagtccaggactgtttcagctgaaccagagggcacacaatttgcatcactgaaactgtcctgggttagtcaatgaaataaaaatgtctaaccacatacacatggatatgatctttgtcggttagattattgataaagtcagtctcagacaagtttccaaactgtgctatttaactagatacaattgagaaattctcaaatgaaaattttatatagtgtcatatcaatcaaaagaaaataatgaaactaagaatacagatcactgttggaagagaaagcagtggtgatggtgtgggtactgcaggaggtggtggggccgtggcacactagaaaagttgggtcacgctgagtaggaagcatttgattttctctggtgcttttagctctggggccggtcaaaggcctctctctggcatggctgtccagggtttgtcccaatgtgtctgagtgagccagcttgagaaggggtcgtgccgtttcttctttcacacaggggaaaaaaaagaccaaacacggaggtgcccagggtgtggatctgctggtgtcccgggagaaccagctggctgggcagcccttcttccccacaggcagctgctattgcgtagggaccgccaggtcaccgagtggccatcacaacaaaccccagcacagtccagcccggccacagccgcctccttgtgtttctgttgtcttccctgctgctgcccacatcctttacccaccgtgtctctcggcccactggaggtatcagaaattccaaattttcaaagcagtttcagtattttcagtatatatgttgggattttataatggttcatggccagaaaaggttcagcacctcccacacacagacattggtccgtttcctgttcttggcatctctgtactttgttggtccaactcagacagcaactttaagatgttcagcgcagccatatcatggcaggactccacatccttgccgataccatggctgatcagaggtggctgagaggagcaattgataagagatacaaattcgttcttgttgtttttggggaagtctttgtattcaacctggaatccctggactctggaaagatagtccagttgctcagagggtctcgtgagaggtccatggggtacgtggcctgaagagatgttattctttaaaatggtctcggctgtgggcgaggtgcccccatacaacaactctcgggctatcatggcagttaccgtggccttggcaggattcggagctgccctggtaaaatctttggtgtgatgtccttgactaactcctacagcctgggcgacctcgggcaccatgggaagaattccagcaggcagctgctgatgacttagataaggcatcctgaactcatcctctttattactagtcccattttcatccccagagccaggttcaaaaaaggttacttttcttccatcccctggtttctttatgggtgtcttctcctctgacttgagtgcgggtttggtgggctgcgcctgcgggactttgaaaccaaggatctccagcatgttctcggctgcattgcgcttggccaccttcttgttggtgcccgttccttctgcagtgtggtttccaaccttcacctgcatcacaaactccctgcggcgcgggaggcctcgctctgtgaggagcgtgtactctggctccttctccttttttgcctgctggatctgggccagtcggctaatcggattgatcccctggccatattctgggcttgtctgtggcttgactatgggttttgttttctttttgattctaggctttactcgttcaactgcaggcaggggcggtaacttcttcagctcctcaagaacagctatggcggcatttttctttgaaatcttcttgcttttcccttcaccttcccccacaaactccccaaccgaaaccttggtcacaaagttcttcatgtggggtgggccactctcccgggccacctgtttcagagggaaagactcgaaattcacaggcaagttccgtttaagtgcaatctcaaacacttgacttatttcagatttattgagattttcttcttcggattctcttccattcacctccagcctctctggcaggggctcattctgcaggatcctcaacgctttggcagcagcatcgtgtttcgcagcctgtcttgtctttcctttgccattaaattgctgtcctcccacagaaagttccacttgataaagtaaaggtggaactggaaatgggtaaaagtacctcgggggataagcacctcctctcatgttgtagttataggtggactgcatccgagagtaagggtcaacaggcttatacattggtttttttccaagtttcatgcacagtgcatttagttctacagtaggggttatgctttctgcagctgcactggtggatgtaatagatgcagagggtaaagcagagttttgaatgggtctacctgcattttcagagggcagagagctagtagtagaaggaatactcatcaaaggctgtgagagaagagactggttcttgttcagtatttggctccctgagagagcagcagatgggttctgaacttgcacttgaacttgagacatggtcactttcaacaaaagtgaacaaatgcaggtaaacagctttcagtgcaggttaattcagtgctatgaagtctaaagttctaccttttttaaaaagagggcgttccaggaacaatgttgtctttgttcagttctgagaggttaagtggttaataaactctggctgctgctccgagctcgtcccccggccggcggtcctgggcggtggcggcgaggaggggaaggaagaaggaaaaaagggagaggaagaagggacgaagggagggaagaggcggagtggccgtggaggaggcgggcgccgccgggccgggggggggaggcggtcaaaggaagcgggagccgagagagacgcggcagccgccggcgcaaacgctgaag

SEQ ID NO: 9340 - RNA, 3210 nt, Homo sapiens
  source 1..3210: mol_type = other RNA
agctggtaaaatggaaccaaatgatcatctaaagtttaaaattcctaaattgtccaatttatacaactgtgggagacttattcaaggtttttgaaagtccaggactgtttcagctgaaccagagggcacacaatttgcatcactgaaactgtcctgggttagtcaatgaaataaaaatgtctaaccacatacacatggatatgatctttgtcggttagattattgataaagtcagtctcagacaagtttccaaactgtgctatttaactagatacaattgagaaattctcaaatgaaaattttatatagtgtcatatcaatcaaaagaaaataatgaaactaagaatacagatcactgttggaagagaaagcagtggtgatggtgtgggtactgcaggaggtggtggggccgtggcacactagaaaagttgggtcacgctgagtaggaagcatttgattttctctggtgcttttagctctggggccggtcaaaggcctctctctggcatggctgtccagggtttgtcccaatgtgtctgagtgagccagcttgagaaggggtcgtgccgtttcttctttcacacaggggaaaaaaaagaccaaacacggaggtgcccagggtgtggatctgctggtgtcccgggagaaccagctggctgggcagcccttcttccccacaggcagctgctattgcgtagggaccgccaggtcaccgagtggccatcacaacaaaccccagcacagtccagcccggccacagccgcctccttgtgtttctgttgtcttccctgctgctgcccacatcctttacccaccgtgtctctcggcccactggaggtatcagaaattccaaattttcaaagcagtttcagtattttcagtatatatgttgggattttataatggttcatggccagaaaaggttcagcacctcccacacacagacattggtccgtttcctgttcttggcatctctgtactttgttggtccaactcagacagcaactttaagatgttcagcgcagccatatcatggcaggactccacatccttgccgataccatggctgatcagaggtggctgagaggagcaattgataagagatacaaattcgttcttgttgtttttggggaagtctttgtattcaacctggaatccctggactctggaaagatagtccagttgctcagagggtctcgtgagaggtccatggggtacgtggcctgaagagatgttattctttaaaatggtctcggctgtgggcgaggtgcccccatacaacaactctcgggctatcatggcagttaccgtggccttggcaggattcggagctgccctggtaaaatctttggtgtgatgtccttgactaactcctacagcctgggcgacctcgggcaccatgggaagaattccagcaggcagctgctgatgacttagataaggcatcctgaactcatcctctttattactagtcccattttcatccccagagccaggttcaaaaaaggttacttttcttccatcccctggtttctttatgggtgtcttctcctctgacttgagtgcgggtttggtgggctgcgcctgcgggactttgaaaccaaggatctccagcatgttctcggctgcattgcgcttggccaccttcttgttggtgcccgttccttctgcagtgtggtttccaaccttcacctgcatcacaaactccctgcggcgcgggaggcctcgctctgtgaggagcgtgtactctggctccttctccttttttgcctgctggatctgggccagtcggctaatcggattgatcccctggccatattctgggcttgtctgtggcttgactatgggttttgttttctttttgattctaggctttactcgttcaactgcaggcaggggcggtaacttcttcagctcctcaagaacagctatggcggcatttttctttgaaatcttcttgcttttcccttcaccttcccccacaaactccccaaccgaaaccttggtcacaaagttcttcatgtggggtgggccactctcccgggccacctgtttcagagggaaagactcgaaattcacaggcaagttccgtttaagtgcaatctcaaacacttgacttatttcagatttattgagattttcttcttcggattctcttccattcacctccagcctctctggcaggggctcattctgcaggatcctcaacgctttggcagcagcatcgtgtttcgcagcctgtcttgtctttcctttgccattaaattgctgtcctcccacagaaagttccacttgataaagtaaaggtggaactggaaatgggtaaaagtacctcgggggataagcacctcctctcatgttgtagttataggtggactgcatccgagagtaagggtcaacaggcttatacattggtttttttccaagtttcatgcacagtgcatttagttctacagtaggggttatgctttctgcagctgcactggtggatgtaatagatgcagagggtaaagcagagttttgaatgggtctacctgcattttcagagggcagagagctagtagtagaaggaatactcatcaaaggctgtgagagaagagactggttcttgttcagtatttggctccctgagagagcagcagatgggttctgaacttgcacttgaacttgagacatggtcactttcaacaaaagtgaacaaatgcaggtaaacagctttcagtgcaggttaattcagtgctatgaagtctaaagttctaccttttttaaaaagagggcgttccaggaacaatgttgtctttgttcagttctgagaggttaagtggttaataaactctgtaatctcagcttatcgggaggctgaagtgggaaaatcgcttgaacctgggaggtggaggttgcagtgagccgagatcacgccactgcactccagcctgggcgacaagagcaaaactccacctggctgctgctccgagctcgtcccccggccggcggtcctgggcggtggcggcgaggaggggaaggaagaaggaaaaaagggagaggaagaagggacgaagggagggaagaggcggagtggccgtggaggaggcgggcgccgccgggccgggggggggaggcggtcaaaggaagcgggagccgagagagacgcggcagccgccggcgcaaacgctgaagagccgctcaggcgcccgcagcccggcaggaagt

SEQ ID NO: 9341 - RNA, 2690 nt, Homo sapiens
  source 1..2690: mol_type = other RNA
agctggtaaaatggaaccaaatgatcatctaaagtttaaaattcctaaattgtccaatttatacaactgtgggagacttattcaaggtttttgaaagtccaggactgtttcagctgaaccagagggcacacaatttgcatcactgaaactgtcctgggttagtcaatgaaataaaaatgtctaaccacatacacatggatatgatctttgtcggttagattattgataaagtcagtctcagacaagtttccaaactgtgctatttaactagatacaattgagaaattctcaaatgaaaattttatatagtgtcatatcaatcaaaagaaaataatgaaactaagaatacagatcactgttggaagagaaagcagtggtgatggtgtgggtactgcaggaggtggtggggccgtggcacactagaaaagttgggtcacgctgagtaggaagcatttgattttctctggtgcttttagctctggggccggtcaaaggcctctctctggcatggctgtccagggtttgtcccaatgtgtctgagtgagccagcttgagaaggggtcgtgccgtttcttctttcacacaggggaaaaaaaagaccaaacacggaggtgcccagggtgtggatctgctggtgtcccgggagaaccagctggctgggcagcccttcttccccacaggcagctgctattgcgtagggaccgccaggtcaccgagtggccatcacaacaaaccccagcacagtccagcccggccacagccgcctccttgtgtttctgttgtcttccctgctgctgcccacatcctttacccaccgtgtctctcggcccactggaggtatcagaaattccaaattttcaaagcagtttcagtattttcagtatatatgttgggattttataatggttcatggccagaaaaggttcagcacctcccacacacagacattggtccgtttcctgttcttggcatctctgtactttgttggtccaactcagacagcaactttaagatgttcagcgcagccatatcatggcaggactccacatccttgccgataccatggctgatcagaggtggctgagaggagcaattgataagagatacaaattcgttcttgttgtttttggggaagtctttgtattcaacctggaatccctggactctggaaagatagtccagttgctcagagggtctcgtgagaggtccatggggtacgtggcctgaagagatgttattctttaaaatggtctcggctgtgggcgaggtgcccccatacaacaactctcgggctatcatggcagttaccgtggccttggcaggattcggagctgccctggtaaaatctttggtgtgatgtccttgactaactcctacagcctgggcgacctcgggcaccatgggaagaattccagcaggcagctgctgatgacttagataaggcatcctgaactcatcctctttattactagtcccattttcatccccagagccaggttcaaaaaaggttacttttcttccatcccctggtttctttatgggtgtcttctcctctgacttgagtgcgggtttggtgggctgcgcctgcgggactttgaaaccaaggatctccagcatgttctcggctgcattgcgcttggccaccttcttgttggtgcccgttccttctgcagtgtggtttccaaccttcacctgcatcacaaactccctgcggcgcgggaggcctcgctctgtgaggagcgtgtactctggctccttctccttttttgcctgctggatctgggccagtcggctaatcggattgatcccctggccatattctgggcttgtctgtggcttgactatgggttttgttttctttttgattctaggctttactcgttcaactgcaggcaggggcggtaacttcttcagctcctcaagaacagctatggcggcatttttctttgaaatcttcttgcttttcccttcaccttcccccacaaactccccaaccgaaaccttggtcacaaagttcttcatgtggggtgggccactctcccgggccacctgtttcagagggaaagactcgaaattcacaggcaagttccgtttaagtgcaatctcaaacacttgacttatttcagatttattgagattttcttcttcggattctcttccattcacctccagcctctctggcaggggctcattctgcaggatcctcaacgctttggcagcagcatcgtgtttcgcagcctgtcttgtctttcctttgccattaaattgctgtcctcccacagaaagttccacttgataaagtaaaggtggaactggaaatgggtaaaagtacctcgggggataagcacctcctctcatgttgtagttataggtggactgcatccgagagtaagggtcaacaggcttatacattggtttttttccaagtttcatgcacagtgcatttagttctacagtaggggttatgctttctggctgctgctccgagctcgtcccccggccggcggtcctgggcggtggcggcgaggaggggaaggaagaaggaaaaaagggagaggaagaagggacgaagggagggaagaggcggagtggccgtggaggaggcgggcgccgccgggccgggggggggaggcggtcaaaggaagcgggagccgagagagacgcggcagccgccggcgcaaacgctgaag

SEQ ID NO: 9342 - RNA, 3323 nt, Homo sapiens
  source 1..3323: mol_type = other RNA
agctggtaaaatggaaccaaatgatcatctaaagtttaaaattcctaaattgtccaatttatacaactgtgggagacttattcaaggtttttgaaagtccaggactgtttcagctgaaccagagggcacacaatttgcatcactgaaactgtcctgggttagtcaatgaaataaaaatgtctaaccacatacacatggatatgatctttgtcggttagattattgataaagtcagtctcagacaagtttccaaactgtgctatttaactagatacaattgagaaattctcaaatgaaaattttatatagtgtcatatcaatcaaaagaaaataatgaaactaagaatacagatcactgttggaagagaaagcagtggtgatggtgtgggtactgcaggaggtggtggggccgtggcacactagaaaagttgggtcacgctgagtaggaagcatttgattttctctggtgcttttagctctggggccggtcaaaggcctctctctggcatggctgtccagggtttgtcccaatgtgtctgagtgagccagcttgagaaggggtcgtgccgtttcttctttcacacaggggaaaaaaaagaccaaacacggaggtgcccagggtgtggatctgctggtgtcccgggagaaccagctggctgggcagcccttcttccccacaggcagctgctattgcgtagggaccgccaggtcaccgagtggccatcacaacaaaccccagcacagtccagcccggccacagccgcctccttgtgtttctgttgtcttccctgctgctgcccacatcctttacccaccgtgtctctcggcccactggaggtatcagaaattccaaattttcaaagcagtttcagtattttcagtatatatgttgggattttataatggttcatggccagaaaaggttcagcacctcccacacacagacattggtccgtttcctgttcttggcatctctgtactttgttggtccaactcagacagcaactttaagatgttcagcgcagccatatcatggcaggactccacatccttgccgataccatggctgatcagaggtggctgagaggagcaattgataagagatacaaattcgttcttgttgtttttggggaagtctttgtattcaacctggaatccctggactctggaaagatagtccagttgctcagagggtctcgtgagaggtccatggggtacgtggcctgaagagatgttattctttaaaatggtctcggctgtgggcgaggtgcccccatacaacaactctcgggctatcatggcagttaccgtggccttggcaggattcggagctgccctggtaaaatctttggtgtgatgtccttgactaactcctacagcctgggcgacctcgggcaccatgggaagaattccagcaggcagctgctgatgacttagataaggcatcctgaactcatcctctttattactagtcccattttcatccccagagccaggttcaaaaaaggttacttttcttccatcccctggtttctttatgggtgtcttctcctctgacttgagtgcgggtttggtgggctgcgcctgcgggactttgaaaccaaggatctccagcatgttctcggctgcattgcgcttggccaccttcttgttggtgcccgttccttctgcagtgtggtttccaaccttcacctgcatcacaaactccctgcggcgcgggaggcctcgctctgtgaggagcgtgtactctggctccttctccttttttgcctgctggatctgggccagtcggctaatcggattgatcccctggccatattctgggcttgtctgtggcttgactatgggttttgttttctttttgattctaggctttactcgttcaactgcaggcaggggcggtaacttcttcagctcctcaagaacagctatggcggcatttttctttgaaatcttcttgcttttcccttcaccttcccccacaaactccccaaccgaaaccttggtcacaaagttcttcatgtggggtgggccactctcccgggccacctgtttcagagggaaagactcgaaattcacaggcaagttccgtttaagtgcaatctcaaacacttgacttatttcagatttattgagattttcttcttcggattctcttccattcacctccagcctctctggcaggggctcattctgcaggatcctcaacgctttggcagcagcatcgtgtttcgcagcctgtcttgtctttcctttgccattaaattgctgtcctcccacagaaagttccacttgataaagtaaaggtggaactggaaatgggtaaaagtacctcgggggataagcacctcctctcatgttgtagttataggtggactgcatccgagagtaagggtcaacaggcttatacattggtttttttccaagtttcatgcacagtgcatttagttctacagtaggggttatgctttcttcatagctgatttttcttgtaggtcttacttttaggattccctcagtgcacggcttccacccccttgacacttcacacatcaggacatcaggggtctcctttattatatgttctgcagtccatcaggctactcatttaagtacaaacaacagcatgaactcaaaaccctggcaggcaggaaggtcaaatggcagaagcctgcaacgcagtacaatccctgggtcatcttggtgattgtctcatggataaatgctgaaggggaaaaagctgcagctgcactggtggatgtaatagatgcagagggtaaagcagagttttgaatgggtctacctgcattttcagagggcagagagctagtagtagaaggaatactcatcaaaggctgtgagagaagagactggttcttgttcagtatttggctccctgagagagcagcagatgggttctgaacttgcacttgaacttgagacatggtcactttcaacaaaagtgaacaaatgcaggtaaacagctttcagtgcaggttaattcagtgctatgaagtctaaagttctaccttttttaaaaagagggcgttccaggaacaatgttgtctttgttcagttctgagaggttaagtggttaataaactctggctgctgctccgagctcgtcccccggccggcggtcctgggcggtggcggcgaggaggggaaggaagaaggaaaaaagggagaggaagaagggacgaagggagggaagaggcggagtggccgtggaggaggcgggcgccgccgggccgggggggggaggcggtcaaaggaagcgggagccgagagagacgcggcagccgccggcgcaaacgctgaag

SEQ ID NO: 9343 - RNA, 3034 nt, Homo sapiens
  source 1..3034: mol_type = other RNA
agctggtaaaatggaaccaaatgatcatctaaagtttaaaattcctaaattgtccaatttatacaactgtgggagacttattcaaggtttttgaaagtccaggactgtttcagctgaaccagagggcacacaatttgcatcactgaaactgtcctgggttagtcaatgaaataaaaatgtctaaccacatacacatggatatgatctttgtcggttagattattgataaagtcagtctcagacaagtttccaaactgtgctatttaactagatacaattgagaaattctcaaatgaaaattttatatagtgtcatatcaatcaaaagaaaataatgaaactaagaatacagatcactgttggaagagaaagcagtggtgatggtgtgggtactgcaggaggtggtggggccgtggcacactagaaaagttgggtcacgctgagtaggaagcatttgattttctctggtgcttttagctctggggccggtcaaaggcctctctctggcatggctgtccagggtttgtcccaatgtgtctgagtgagccagcttgagaaggggtcgtgccgtttcttctttcacacaggggaaaaaaaagaccaaacacggaggtgcccagggtgtggatctgctggtgtcccgggagaaccagctggctgggcagcccttcttccccacaggcagctgctattgcgtagggaccgccaggtcaccgagtggccatcacaacaaaccccagcacagtccagcccggccacagccgcctccttgtgtttctgttgtcttccctgctgctgcccacatcctttacccaccgtgtctctcggcccactggaggtatcagaaattccaaattttcaaagcagtttcagtattttcagtatatatgttgggattttataatggttcatggccagaaaaggttcagcacctcccacacacagacattggtccgtttcctgttcttggcatctctgtactttgttggtccaactcagacagcaactttaagatgttcagcgcagccatatcatggcaggactccacatccttgccgataccatggctgatcagaggtggctgagaggagcaattgataagagatacaaattcgttcttgttgtttttggggaagtctttgtattcaacctggaatccctggactctggaaagatagtccagttgctcagagggtctcgtgagaggtccatggggtacgtggcctgaagagatgttattctttaaaatggtctcggctgtgggcgaggtgcccccatacaacaactctcgggctatcatggcagttaccgtggccttggcaggattcggagctgccctggtaaaatctttggtgtgatgtccttgactaactcctacagcctgggcgacctcgggcaccatgggaagaattccagcaggcagctgctgatgacttagataaggcatcctgaactcatcctctttattactagtcccattttcatccccagagccaggttcaaaaaaggttacttttcttccatcccctggtttctttatgggtgtcttctcctctgacttgagtgcgggtttggtgggctgcgcctgcgggactttgaaaccaaggatctccagcatgttctcggctgcattgcgcttggccaccttcttgttggtgcccgttccttctgcagtgtggtttccaaccttcacctgcatcacaaactccctgcggcgcgggaggcctcgctctgtgaggagcgtgtactctggctccttctccttttttgcctgctggatctgggccagtcggctaatcggattgatcccctggccatattctgggcttgtctgtggcttgactatgggttttgttttctttttgattctaggctttactcgttcaactgcaggcaggggcggtaacttcttcagctcctcaagaacagctatggcggcatttttctttgaaatcttcttgcttttcccttcaccttcccccacaaactccccaaccgaaaccttggtcacaaagttcttcatgtggggtgggccactctcccgggccacctgtttcagagggaaagactcgaaattcacaggcaagttccgtttaagtgcaatctcaaacacttgacttatttcagatttattgagattttcttcttcggattctcttccattcacctccagcctctctggcaggggctcattctgcaggatcctcaacgctttggcagcagcatcgtgtttcgcagcctgtcttgtctttcctttgccattaaattgctgtcctcccacagaaagttccacttgataaagtaaaggtggaactggaaatgggtaaaagtacctcgggggataagcacctcctctcatgttgtagttataggtggactgcatccgagagtaagggtcaacaggcttatacattggtttttttccaagtttcatgcacagtgcatttagttctacagtaggggttatgctttcttcatagctgatttttcttgtaggtcttacttttaggattccctcagtgcacggcttccacccccttgacacttcacacatcaggacatcaggggtctcctttattatatgttctgcagtccatcaggctactcatttaagtacaaacaacagcatgaactcaaaaccctggcaggcaggaaggtcaaatggcagaagcctgcaacgcagtacaatccctgggtcatcttggtgattgtctcatggataaatgctgaaggggaaaaagcttttttaaaaagagggcgttccaggaacaatgttgtctttgttcagttctgagaggttaagtggttaataaactctggctgctgctccgagctcgtcccccggccggcggtcctgggcggtggcggcgaggaggggaaggaagaaggaaaaaagggagaggaagaagggacgaagggagggaagaggcggagtggccgtggaggaggcgggcgccgccgggccgggggggggaggcggtcaaaggaagcgggagccgagagagacgcggcagccgccggcgcaaacgctgaag

SEQ ID NO: 9344 - RNA, 2765 nt, Homo sapiens
  source 1..2765: mol_type = other RNA
agctggtaaaatggaaccaaatgatcatctaaagtttaaaattcctaaattgtccaatttatacaactgtgggagacttattcaaggtttttgaaagtccaggactgtttcagctgaaccagagggcacacaatttgcatcactgaaactgtcctgggttagtcaatgaaataaaaatgtctaaccacatacacatggatatgatctttgtcggttagattattgataaagtcagtctcagacaagtttccaaactgtgctatttaactagatacaattgagaaattctcaaatgaaaattttatatagtgtcatatcaatcaaaagaaaataatgaaactaagaatacagatcactgttggaagagaaagcagtggtgatggtgtgggtactgcaggaggtggtggggccgtggcacactagaaaagttgggtcacgctgagtaggaagcatttgattttctctggtgcttttagctctggggccggtcaaaggcctctctctggcatggctgtccagggtttgtcccaatgtgtctgagtgagccagcttgagaaggggtcgtgccgtttcttctttcacacaggggaaaaaaaagaccaaacacggaggtgcccagggtgtggatctgctggtgtcccgggagaaccagctggctgggcagcccttcttccccacaggcagctgctattgcgtagggaccgccaggtcaccgagtggccatcacaacaaaccccagcacagtccagcccggccacagccgcctccttgtgtttctgttgtcttccctgctgctgcccacatcctttacccaccgtgtctctcggcccactggaggtatcagaaattccaaattttcaaagcagtttcagtattttcagtatatatgttgggattttataatggttcatggccagaaaaggttcagcacctcccacacacagacattggtccgtttcctgttcttggcatctctgtactttgttggtccaactcagacagcaactttaagatgttcagcgcagccatatcatggcaggactccacatccttgccgataccatggctgatcagaggtggctgagaggagcaattgataagagatacaaattcgttcttgttgtttttggggaagtctttgtattcaacctggaatccctggactctggaaagatagtccagttgctcagagggtctcgtgagaggtccatggggtacgtggcctgaagagatgttattctttaaaatggtctcggctgtgggcgaggtgcccccatacaacaactctcgggctatcatggcagttaccgtggccttggcaggattcggagctgccctggtaaaatctttggtgtgatgtccttgactaactcctacagcctgggcgacctcgggcaccatgggaagaattccagcaggcagctgctgatgacttagataaggcatcctgaactcatcctctttattactagtcccattttcatccccagagccaggttcaaaaaaggttacttttcttccatcccctggtttctttatgggtgtcttctcctctgacttgagtgcgggtttggtgggctgcgcctgcgggactttgaaaccaaggatctccagcatgttctcggctgcattgcgcttggccaccttcttgttggtgcccgttccttctgcagtgtggtttccaaccttcacctgcatcacaaactccctgcggcgcgggaggcctcgctctgtgaggagcgtgtactctggctccttctccttttttgcctgctggatctgggccagtcggctaatcggattgatcccctggccatattctgggcttgtctgtggcttgactatgggttttgttttctttttgattctaggctttactcgttcaactgcaggcaggggcggtaacttcttcagctcctcaagaacagctatggcggcatttttctttgaaatcttcttgcttttcccttcaccttcccccacaaactccccaaccgaaaccttggtcacaaagttcttcatgtggggtgggccactctcccgggccacctgtttcagagggaaagactcgaaattcacaggcaagttccgtttaagtgcaatctcaaacacttgacttatttcagatttattgagattttcttcttcggattctcttccattcacctccagcctctctggcaggggctcattctgcaggatcctcaacgctttggcagcagcatcgtgtttcgcagcctgtcttgtctttcctttgccattaaattgctgtcctcccacagaaagttccacttgataaagtaaaggtggaactggaaatgggtaaaagtacctcgggggataagcacctcctctcatgttgtagttataggtggactgcatccgagagtaagggtcaacaggcttatacattggtttttttccaagtttcatgcacagtgcatttagttctacagtaggggttatgctttcttttttaaaaagagggcgttccaggaacaatgttgtctttgttcagttctgagaggttaagtggttaataaactctggctgctgctccgagctcgtcccccggccggcggtcctgggcggtggcggcgaggaggggaaggaagaaggaaaaaagggagaggaagaagggacgaagggagggaagaggcggagtggccgtggaggaggcgggcgccgccgggccgggggggggaggcggtcaaaggaagcgggagccgagagagacgcggcagccgccggcgcaaacgctgaag

SEQ ID NO: 9345 - RNA, 2888 nt, Homo sapiens
  source 1..2888: mol_type = other RNA
agctggtaaaatggaaccaaatgatcatctaaagtttaaaattcctaaattgtccaatttatacaactgtgggagacttattcaaggtttttgaaagtccaggactgtttcagctgaaccagagggcacacaatttgcatcactgaaactgtcctgggttagtcaatgaaataaaaatgtctaaccacatacacatggatatgatctttgtcggttagattattgataaagtcagtctcagacaagtttccaaactgtgctatttaactagatacaattgagaaattctcaaatgaaaattttatatagtgtcatatcaatcaaaagaaaataatgaaactaagaatacagatcactgttggaagagaaagcagtggtgatggtgtgggtactgcaggaggtggtggggccgtggcacactagaaaagttgggtcacgctgagtaggaagcatttgattttctctggtgcttttagctctggggccggtcaaaggcctctctctggcatggctgtccagggtttgtcccaatgtgtctgagtgagccagcttgagaaggggtcgtgccgtttcttctttcacacaggggaaaaaaaagaccaaacacggaggtgcccagggtgtggatctgctggtgtcccgggagaaccagctggctgggcagcccttcttccccacaggcagctgctattgcgtagggaccgccaggtcaccgagtggccatcacaacaaaccccagcacagtccagcccggccacagccgcctccttgtgtttctgttgtcttccctgctgctgcccacatcctttacccaccgtgtctctcggcccactggaggtatcagaaattccaaattttcaaagcagtttcagtattttcagtatatatgttgggattttataatggttcatggccagaaaaggttcagcacctcccacacacagacattggtccgtttcctgttcttggcatctctgtactttgttggtccaactcagacagcaactttaagatgttcagcgcagccatatcatggcaggactccacatccttgccgataccatggctgatcagaggtggctgagaggagcaattgataagagatacaaattcgttcttgttgtttttggggaagtctttgtattcaacctggaatccctggactctggaaagatagtccagttgctcagagggtctcgtgagaggtccatggggtacgtggcctgaagagatgttattctttaaaatggtctcggctgtgggcgaggtgcccccatacaacaactctcgggctatcatggcagttaccgtggccttggcaggattcggagctgccctggtaaaatctttggtgtgatgtccttgactaactcctacagcctgggcgacctcgggcaccatgggaagaattccagcaggcagctgctgatgacttagataaggcatcctgaactcatcctctttattactagtcccattttcatccccagagccaggttcaaaaaaggttacttttcttccatcccctggtttctttatgggtgtcttctcctctgacttgagtgcgggtttggtgggctgcgcctgcgggactttgaaaccaaggatctccagcatgttctcggctgcattgcgcttggccaccttcttgttggtgcccgttccttctgcagtgtggtttccaaccttcacctgcatcacaaactccctgcggcgcgggaggcctcgctctgtgaggagcgtgtactctggctccttctccttttttgcctgctggatctgggccagtcggctaatcggattgatcccctggccatattctgggcttgtctgtggcttgactatgggttttgttttctttttgattctaggctttactcgttcaactgcaggcaggggcggtaacttcttcagctcctcaagaacagctatggcggcatttttctttgaaatcttcttgcttttcccttcaccttcccccacaaactccccaaccgaaaccttggtcacaaagttcttcatgtggggtgggccactctcccgggccacctgtttcagagggaaagactcgaaattcacaggcaagttccgtttaagtgcaatctcaaacacttgacttatttcagatttattgagattttcttcttcggattctcttccattcacctccagcctctctggcaggggctcattctgcaggatcctcaacgctttggcagcagcatcgtgtttcgcagcctgtcttgtctttcctttgccattaaattgctgtcctcccacagaaagttccacttgataaagtaaaggtggaactggaaatgggtaaaagtacctcgggggataagcacctcctctcatgttgtagttataggtggactgcatccgagagtaagggtcaacaggcttatacattggtttttttccaagtttcatgcacagtgcatttagttctacagtaggggttatgctttcttttttaaaaagagggcgttccaggaacaatgttgtctttgttcagttctgagaggttaagtggttaataaactctgtaatctcagcttatcgggaggctgaagtgggaaaatcgcttgaacctgggaggtggaggttgcagtgagccgagatcacgccactgcactccagcctgggcgacaagagcaaaactccacctggctgctgctccgagctcgtcccccggccggcggtcctgggcggtggcggcgaggaggggaaggaagaaggaaaaaagggagaggaagaagggacgaagggagggaagaggcggagtggccgtggaggaggcgggcgccgccgggccgggggggggaggcggtcaaaggaagcgggagccgagagagacgcggcagccgccggcgcaaacgctgaag

SEQ ID NO: 9346 - RNA, 2740 nt, Homo sapiens
  source 1..2740: mol_type = other RNA
agctgtctgaaaatgtcttgggaaagttttacaaaaaaaaaaatcaacagaagcaagttatgaaaatatttgaccagcttcatctttggttatttcttattgcagctctgtaaggacagactgttcccaaagctccagccatggcaggaagggaagcaaatcagtccctgtataaaccatttaaccaattgaatgtatcacatgttgataaatacatagaagcaggccctagggcctacaaaaccagccccactcccaaccacaaggttgaaagtcttatggggcagaacattaagactcctttataaatatgaaaatagattaatcaacaggaaaaggtctttgaataggttagctaagagccatgaccaccacgctgccttgctgtccccttgcatagaaatgtagtgacgtggtctgaccatgcagtaagtgcaaacagcaattactcaaatgtcttagaatactggcaagaagcaccccaatattcaggtctgggaaacagccatgaccattacggcctcttgatcagctccatgttccactcagtagcttatatgccccaagaaaaggcaagagacagacctggggtggggaaagaaccggggtaatagctgcctgccagctcagcctagaactagacatcctctggtcctatctggggaagtacactggagagggtctggtgggaggcagacctccttgctggatttcagaggcttggtatcagctgttggccctaactaggaaggcctctcactgctgcctcccgtcatacacagccaatgggcactgggagcccagaagttgagcctggcttggcctagcctgcctgctctgtaggctccagggaagaatcaaggctgtgcacctagggggccatatggtttcagctgaaggtccatccccaaggtgaggcagggactaaaccccctcacccatcctgctttccctgggtttgcaggcctatgcctgaggtggagaaggtggctggagttgagcctgctggcctttcttctacctccatctcctcagaagcacccgcagggcatggactggtcccctggggcctggacccaaaaccattttcttcctggagaatggagcagtccatagcctcatgggcttgagcagctggtagggcagatgcccggaatggtgggatctctttaactctgtacttgagactacttaggcgtggtgggggcccatcagatagcgattcttcccggcccacaaatggacaagcctcttgatgcaagaactcaggcgaaccaggcaaggaacgccaccggcgaataggtggggccaggggctcctgccagtcagccaggggcatagttccgggccctggtgcatccaggtcaaataccagagagatgacagacttgctgggcaggtcaaaaaacttgatcttgccccccatgaggtcctggcgagcactaaaagggttgactttgggggtgcgggcagcaccatctcgtggccggtagtatgggtccaagacactcactgtacgtgggggcttacgggaaaagatatctgactggcttcgagacagccagatggtacgtcttgggcatggtgacttgtgggggatcttgtcatccagtgagcttagtcgcttcaccccaggtgctttctccaagagtcccctggctgtgggctgcagcttcctatccctctcctgctcttcttcctgtaggcggctcagaatttcctccagggtcttcccaatctccacaaaagatgggcgcagtttgggatccatgttacagcagttgaaagtaagttgcagaaaatctgggggacagtctcccaccatgtgctggaaagcatcatagtccagcccgaaattctctgtgcggggaagatagtccggatcggcctggatgcgggcgatgatctcgcagaggatgataccataagagaacacatctgccttttcattatagggctcatctcggagaacctcaggtgccatccagaatggggaacccaccacggccagcttctcactccccatgctgacatcggggatcttctcagccaggccaaagtcagctaccactgcagagtaaccattctcatccctctttatcaggcagttcttagatgtgaggtcccgatgaaaaatgcctttgaagtgaaggtagctgaggcccactgctatgtcataggccagttttaccctcacagtccaaggcaaatgcaggttactgtctagcaactgttccaggttcccggagttgatatactctgtaagtgcatgcaattgtccttgatgaacacatacacccatgaacctaaggatgttgggatgggagagtctattcatgagctgtacttctttcagcatgtttgcccggttactgctcaatgtgttcatcttaagagccatcacctgaccagaagctcggtgtcgtacctgaggcaggactgagcagccagaggggtgcctgcgcgggcaagaggaggagacggcggcaaagagggagcatagtaaccctcacagctcgttggtggcagcggctccttagcctgcggaggcggtgggagcccctagcgcagaagccggcgactcagctaggctagcggcggcggcgaacgaggagactactgccatggccccacagtcggggccgctccccccgcctgtttggcggggccaggaggacgatccgaccagcgaagccaacagggcagctggtagctctgctgagctcccgggccgcgaaag

SEQ ID NO: 9347 - RNA, 3048 nt, Homo sapiens
  source 1..3048: mol_type = other RNA
agctgtctgaaaatgtcttgggaaagttttacaaaaaaaaaaatcaacagaagcaagttatgaaaatatttgaccagcttcatctttggttatttcttattgcagctctgtaaggacagactgttcccaaagctccagccatggcaggaagggaagcaaatcagtccctgtataaaccatttaaccaattgaatgtatcacatgttgataaatacatagaagcaggccctagggcctacaaaaccagccccactcccaaccacaaggttgaaagtcttatggggcagaacattaagactcctttataaatatgaaaatagattaatcaacaggaaaaggtctttgaataggttagctaagagccatgaccaccacgctgccttgctgtccccttgcatagaaatgtagtgacgtggtctgaccatgcagtaagtgcaaacagcaattactcaaatgtcttagaatactggcaagaagcaccccaatattcaggtctgggaaacagccatgaccattacggcctcttgatcagctccatgttccactcagtagcttatatgccccaagaaaaggcaagagacagacctggggtggggaaagaaccggggtaatagctgcctgccagctcagcctagaactagacatcctctggtcctatctggggaagtacactggagagggtctggtgggaggcagacctccttgctggatttcagaggcttggtatcagctgttggccctaactaggaaggcctctcactgctgcctcccgtcatacacagccaatgggcactgggagcccagaagttgagcctggcttggcctagcctgcctgctctgtaggctccagggaagaatcaaggctgtgcacctagggggccatatggtttcagctgaaggtccatccccaaggtgaggcagggactaaaccccctcacccatcctgctttccctgggtttgcaggcctatgcctgaggtggagaaggtggctggagttgagcctgctggcctttcttctacctccatctcctcagaagcacccgcagggcatggactggtcccctggggcctggacccaaaaccattttcttcctggagaatggagcagtccatagcctcatgggcttgagcagctggtagggcagatgcccggaatggtgggatctctttaactctgtacttgagactacttaggcgtggtgggggcccatcagatagcgattcttcccggcccacaaatggacaagcctcttgatgcaagaactcaggcgaaccaggcaaggaacgccaccggcgaataggtggggccaggggctcctgccagtcagccaggggcatagttccgggccctggtgcatccaggtcaaataccagagagatgacagacttgctgggcaggtcaaaaaacttgatcttgccccccatgaggtcctggcgagcactaaaagggttgactttgggggtgcgggcagcaccatctcgtggccggtagtatgggtccaagacactcactgtacgtgggggcttacgggaaaagatatctgactggcttcgagacagccagatggtacgtcttgggcatggtgacttgtgggggatcttgtcatccagtgagcttagtcgcttcaccccaggtgctttctccaagagtcccctggctgtgggctgcagcttcctatccctctcctgctcttcttcctgtaggcggctcagaatttcctccagggtcttcccaatctccacaaaagatgggcgcagtttgggatccatgttacagcagttgaaagtaagttgcagaaaatctgggggacagtctcccaccatgtgctggaaagcatcatagtccagcccgaaattctctgtgcggggaagatagtccggatcggcctggatgcgggcgatgatctcgcagaggatgataccataagagaacacatctgccttttcattatagggctcatctcggagaacctcaggtgccatccagaatggggaacccaccacggccagcttctcactccccatgctgacatcggggatcttctcagccaggccaaagtcagctaccactgcagagtaaccattctcatccctctttatcaggcagttcttagatgtgaggtcccgatgaaaaatgcctttgaagtgaaggtagctgaggcccactgctatgtcataggccagttttaccctcacagtccaaggcaaatgcaggttactgtctagcaactgttccaggttcccggagttgatatactctgtaagtgcatgcaattgtccttgatgaacacatacacccatgaacctaaggatgttgggatgggagagtctattcatgagctgtacttctttcagcatgtttgcccggttactgctcaatgtgttcatcttaagagccatcacctgaccagaagctcggtgtcgtaccttgaacacttcagaaaagaagccagaccctattttttcacaggtgaaatcatccaaacgcgtcagtctggaaaaggcacttataagagctcgatacgaagatggccaaactcttcccacctggctcacatttccttctcctccaccacctccttcaaactcttcaagacgctccacacgtggaggaaatcctgcaattgaattccgtttgctccgatccatagtctaaataatcacttttttcttcttttaagaaggaactccacacataaatttttgttgaattttacttctcttctggtttgacactgaggcaggactgagcagccagaggggtgcctgcgcgggcaagaggaggagacggcggcaaagagggagcatagtaaccctcacagctcgttggtggcagcggctccttagcctgcggaggcggtgggagcccctagcgcagaagccggcgactcagctaggctagcggcggcggcgaacgaggagactactgccatggccccacagtcggggccgctccccccgcctgtttggcggggccaggaggacgatccgaccagcgaagccaacagggcagctggtagctctgctgagctcccgggccgcgaaag

SEQ ID NO: 9348 - RNA, 2689 nt, Homo sapiens
  source 1..2689: mol_type = other RNA
agctgtctgtgttttccttctcagaacttgccattagtagaatgtctctgaaagtcccagcagcttttcaatagaggagacacaaggtagctgtgagatgcagaggccttgatacaaatctcaggagctggtttgccaatgggatcatcaagtttttctccccagcagggacatctcgtgtcatctgttgttctggatggctttggctcaaggtctttcttgaggttgcagtcaagacactgaagctgctgtcatctcaagaccaccagggaccggagcacctgcttccagtatggctcacttaatggctttggatgaaggcctcagttccttgccgttgccagggcacctcagtaccttgccatttgaacactctgtgagactgcttgagtgttttcacagcatggcagctggcctcccctcagagtgagtgatccaaaagagggatcaagagaaaaaacacaatgatttttttaggtattctcaaaatccacacactatcacattcaccatattctgttagaagtaagtcactaagtctagcctccatcaagaggagggcattaggctccaccctttgaaaataggtgtatcaaagaatttatatacatattttcaaaccacaacattaagatttggagatggtggctgctgctttctttgtgtatttgttttggacttatgcttacagtaagcagaagtattctgaagtgaaaaaaatataaatctcaattgcagagaattattttaataaagtgttatgtaataccctttattttcgccacaataattattttaataaaatataatgcaatatgttttattttcagctaaaggacttttatcctttgaagagtgagaaacagagaaactcccaaaaacctgcaccccaaaattataagaatgagaacattttaagataaaaattcctttaatgtttttctctttcaccagtacaaaaagtgatattttaataaagcagcatcaattagagaaactgctaatgtttatacagagttacattcttacattcaaaattactcaggcccaatcttactttctccctaataacaatagtttaatcaaggaggtaatatttaatgcaatctaatatctatcctttctttaaaaattgccacaaacttctcacttaatcaactagcattcacagtacaaaactgagaactaaaaataaaatcctaagcccccaaccaactgaatggacgcccctcttggccaagaggacccagagaaaccttaaaaatggagttcctggccacgacaggacaggaggttggacacacattggtatatctcctctttgtgtggtttagacacaactgatcagcattagtgttaaaatagagttcataagactgataaaatggactctgtagcagtaagataccaaattacaaacaggacctaaggccacccagtcaaggattaagccacatacccctacacttaaagaataaactgtgttctaactgccacaggtttttcttcttctacagaagctaaataagcaaaggccttaagagaagcaatattgaaataattgcagctcctctaccaccagatgctgactcactggtcccctgttccacaagccataactataactttgattggacaagactgatttcagtaactctcctgataaaagaccagagaccatggactggtcccagcccatttaaagagactgcacacttgagtgtcttcatctccctgcttcaccttttgacatataaggcctaactgtaacgcgtttaaatattacggctccacaccaaagtgaacatgggatgcatgaaacatgcatgtttgtttatgtatcaggccccacttcaggaatatctgtagctcctcctataacctgttgaatatgtgtactgggccaacctgtttagcataaatcccagccccacactcccctccctcaaagtgcccccttcaagtccctgccagaggctacacttccaaatctgtcaggatgatggccaccctagaagctgtaaccctttttataataaataaagtctcctttccaaatttatagaacttgggatttttcaattgacaaaacttttgaaatctacataggttgataaaacaaggcaaacaaggacccatgcttattaattggcttcaatttacttcaatattatggaagttcttccacatattatttatattatcttccttttatataatacattttaaaaatcacaagatgaatgagcatttgaatcatgattaaggacatcagaaaaacttctttggggatatgccatatacaactttgatattatctgaagctttttggaaaactcattcaaaaaaattgttttgatgccctcttttttctaagtaaaatcaaaatactggtcattatggtgctcttaaaaatgtctttgttatcaaaactagcatcaacacattgcaatacaatgtcataaaagcccacctgtctttacaattcattaattgaacttctagtttaacgatgtggtttaaatcagaatatcttccttattttcttgggagtgttctgaaggagatcaagtctacagccatgccaccctgaacgtgcctgatcttgtttaaaagagatcaagatgggccaggagcggtggctcacgcctgtaatcccagcactttgggaggccgaggcaggcggatc

SEQ ID NO: 9349 - RNA, 570 nt, Homo sapiens
  source 1..570: mol_type = other RNA
agctgtctgtgttttccttctcagaacttgccattagtagaatgtctctgaaagtcccagcagcttttcaatagaggagacacaaggtagctgtgagatgcagaggccttgatacaaatctcaggagctggtttgccaatgggatcatcaagtttttctccccagcagggacatctcgtgtcatctgttgttctggatggctttggctcaaggtctttcttgaggttgcagtcaagacactgaagctgctgtcatctcaagaccaccagggaccggagcacctgcttccagtatggctcacttaatggctttggatgaaggcctcagttccttgccgttgccagggcacctcagtaccttgccatttgaacactctgtgagactgcttgagtgttttcacagcatggcagctgtctttacaattcattaattgaacttctagtttaacgatgtggtttaaatcagaatatcttccttattttcttgggagtgttcaggatggatgactcaagaggtatcacgtgtccatttgtcctcttgtgctactgccattcatcttgtgcaatggga

SEQ ID NO: 9350 - RNA, 51 nt, Homo sapiens
  source 1..51: mol_type = other RNA
agcttctttacagtgctgccttgcgttctgtggagaagactagagaggacc

SEQ ID NO: 9351 - RNA, 60 nt, Homo sapiens
  source 1..60: mol_type = other RNA
agcttctttacagtgctgccttgtagcattcaggtcaagcagcattgtacagggctatga

SEQ ID NO: 9352 - RNA, 60 nt, Homo sapiens
  source 1..60: mol_type = other RNA
agcttctttacagtgctgccttgttgcatatggatcaagcagcattgtacagggctatga

SEQ ID NO: 9353 - RNA, 672 nt, Homo sapiens
  source 1..672: mol_type = other RNA
aggaaacagggacccagtggcttggtggtttgggaagaacacttggtgatggcggctcactaaatttggcaccagcatagttctgattagcttgagatttaaaaagtaacctgggacctgataagctagaattccaactttgattatttggaaaatttttgttcttccccccattttgcatggcctgccaggcagctgctgatgagttataaccatgtcctctttcttttttcttatgaacaatcttcatctgggaattctgttccttggtcttctgtctgttaagctgttgttggttcttactaacatttctagattgaggggctggaatgttatacctctctccaccacccatcttcagcttctttgtcacctttcagtctgcttttcagattgcaggatctccactacctgtcctcttccttgctgccaagcccaagataacaagtgttgctttctgacagatcccttcctttgtctcaatacagaagttttcatgggccgatctgctgagttcagcctaggagctgaggccaacatctgagtctcctcagcacacaagtttgagagaagtcctagtcaaaagttgcctccctgtgaaggcggttcagacacacgcgggcaagtcagtcacttcctgcttggtggccccattggtccttaagttcaatt

SEQ ID NO: 9354 - RNA, 750 nt, Homo sapiens
  source 1..750: mol_type = other RNA
aggaaacagggacccagtggcttggtggtttgggaagaacacttggtgatggcggctcactaaatttggcaccagcatagttctgattagcttgagatttaaaaagtaacctgggacctgataagctagaattccaactttgattatttggaaaatttttgttcttccccccattttgcatggcctgccaggcagctgctgatgagttataaccatgtcctctttcttttttcttatgaacaatcttcatctgggaattctgttccttggtcttctgtctgttaagctgttgttggttcttactaacatttctagattgaggggctggaatgttatacctctctccaccacccatcttcagcttctttgtcacctttcagtctgcttttcagattgcaggatctccactacctgtcctcttccttgctgccaagcccaagataacaagtgttgctttctgacagatcccttcctttgtctcaatacagaagttttcatgggccgatctgctgagttcagcctaggagctgaggccaacatctgagtctcctcagcacacaagtttgagagaagtcctagtgacttcaagctcggaactaacgcggcagcggctccctctcgacgtcgaagcctccctccctttccagggagagacgaggcacggaccgacaaagcccacgaacaccgatgagcgagctgccggccaccccagcttctacaacccgaccttctccttctgcctctaccgac

SEQ ID NO: 9355 - RNA, 739 nt, Homo sapiens
  source 1..739: mol_type = other RNA
aggaagccctggaggggctggagagtgccacacctgccataccgtagggaaagcaatgtccgttcacatccaggaaacggagatactcgcgaccgagggagccttccggcaggctctggagcttgcccaggtcgagggtggatgtcgaaatccggggacgctcccgtggcggtaggggttatagagcgccatcgccgcggagccggcggccaacagccctttctgcagcggggaggtggggaggtggtgcgagtatagcgggccggcgccgtcgctcctagcccggaggggcatttctgccgcaggccgctgtaggcccgggagcccgcagagccgacggaggacagggcgcagcagagtcgccatggcagcgggcgtccgcggaggatgggcgggtacgaagaacgccgcgattctgtcaggcgacggagcgtcggaggggtcaaaactcactgaaaaaccgattctgacggcgtagcctacggcctttcgaggggaaacatcgcttcacgggcagaaggcatgtaggccaagtaggcgaaggaaacgcacgcgaactgtctaccgtctacgtccaccgatccaagactctcgccatgtcacctcgccccagaaagtgtctgcaaaggacacgcaaccacgctcactcagcgccgggccctatttccttctccacagccggttttccccgaagactataaaatgcgaacctcttccggctgtggaacatggcggcgcc

SEQ ID NO: 9356 - RNA, 8371 nt, Homo sapiens
  source 1..8371: mol_type = other RNA
aggaagccctggaggggctggaggagctggtgtcactggggggcagggtgcagctactgctgtggcctgagccaactgcatcaggtctttttctttcttaattttcaggtctctcttcagctcttcctgcacttcaatttgcagatccttgtccaggagtgctctcttcttcaggatctcggctctgagctgctctttgtgcttgaagagcagagctgacagcttagtggcattctgcttgctacgtttctgctccacactctcttcacgcttccgtttttttgctgcctgtttttcttctttatctatcttatccaaaatatacttcatcacctggttacagacaatcattctttgattctcttctctttcagctggagtcatgctctttttctgttttaaatgttctattacagcattatgcttcatcaccacctggggttgtgactgtggctggccttgggaaggtatctgaagagatgtatgtggttgaattggaatcggttgtgaggttgtagtctgaacctgggattgttgtccaggagacagttgggatggagttgatggacgtattcgagtctgtgatggactttggacacgaacaggagactgtccttggacattactttgaggctgagactgtgctgcaacttggggcttggatgactgtgcgtgggtgggttgtgcttcagaagggacatgggatgaaacagttgtttgggtctgaacttcaggctgagtctgaacttcaggctgagctggggactggggctgggtttggggctggggctgagctgaaggctgagcagtctgtggctgggcttctgctggacccacacttgatgactgagctggtggcagggttttgtcttgatgtacctgcatctggggtgacagtttactctgcctttgttcacctgtacctgctgctgtcgtggaaacagtggtggtggtggtgctggctgtggtggctgttgttgccaatggggtaaagaggaatcgctgaacagtaccatttggcattgcagcttgcattagctgctggcctgggcctgggagtacagtcaccccttgaggtatcaactgcaactgtccagtagtttgaccttgtccttgaattactactgtcaaaccttgattgccaccgtggccctgtgttaactgagtaagttgagccatggtgagcttcacttgtccttgttgggggcgagggggttgtgaggctgaagactgtatatttgaagtggacgttgctgaagttaagcttttctgcccaggtgttgaggaaaccgtgttaggggcggagactgcagtggagacaggctgccccctgatgatttgagtcatcacttgctgaggagcacctggctgtaccatcacaggtgttcgaataattgcctttcctagtgttgactgttggagtggtgttctaatcacggtcataccagggcgaatctgaggccctgtgattacttgtgaattgcttgtggttcctccagagcctgaggtattgggcctaattgtgactgttgctgtcctgggctggaatgaagtaaaggtttgctgactggtacctgtacttgatggaatgatacccaggactttctgctgtacttgaacaacgcctccttgtgttgctggcacatttacagcgacaatcttgctgtttgcaggaagtggcagtttggtaattacttttcctgccatagtgactggattgcctgtaatttggaacgtctgacctgtgctggcaatggttgtagcagatgtggcagctgtgctggtggctgaatttgactggccttgcttaacccatgtagcaaaggtttgatgaaagttcttgttttgttggaatgttactgtagctggagatccaactttagtagttagtaccattttggttccagttgtaactgagccacttatgggggccaccataaccttctgtgctggagagatggtgctggttgtactgcttgttggggaagtagtggaagttgcaatcactgtcggcttctgctgctccagtcgtttcttagcctgttgctcaactgcttgtgccttttctttctccactctctcagcaaatgccctgatctcccacaattccagttcttcttctgctacccaggtttcaataataacagggccagtttgcttgggcgtttctggtctctttggccgcagtgcacttgatcgaaggcctttcctctgaggtgtaggcgtttcttttggtgtttctggaactccaatgggacaaatgattttcctgatacaatattcagatcgaatgccataaggaccaacatctctcctcttaattatttctgttgttgtgatttcagtttcggatgtttctgtccgtgtagtccctcctcctggaggagccttggccgccatatcatcccatctcaaacttgcccacagtaaccgtaacatcaggctcactccagctaaggactttactgtctgaagtctatacctccaagtgatgccaaaggtcggtctaggagaaggatatggccatatatccaaagcaggttttgcattgtaattaaaataagggacctctcggattcctccttttcgggccaacttttttaagtcatcattaggcaaaacaaaaatgctcttcttgctgctcttggtaacaaattttctataggatggcagagctgtacctgaacgagtcttctttggtcttgaaaatttcatcagtttcactttgtctcgtgtggaatactctttgctcacagtcatagatgtaaccagtgtgcctcccgtggtggtcagggagtctgtcactgtcgtggtgaccacggttttgctctgctcctttacagagatgatgtccacactgccgcctgtggagggtgtggaaagcttggtcactgttgtagtggtggttgtgacagtggattttgcacaattttctgtggaagaaaccacagtttgcttatcgcctttttctaccttgatcacagtttttgattctgtggccactgtggaggtcatcgtggtgacttctgtgatgacggtttttcttttagattctccattgacattttcatttttgttgatgggcagaccattttcatcaataaagtcattactgagattagattcctcttcagaagtaataggtgatgaagtaactttcttaacttctgaggtttctatttccatatcttctacctgattaactgaattgctttctggacaagatgctgagggtgtggtcgtctgtgtactgtcagactctttggttgatggcagggtctcaaggctatctcggtagttaccttcagcatctgaagaactcagcaaatgcgattttgtttcggagctgtttctttcattaaaatcttccatgatgacatcaccattaatgaatggccttatagcagattctttaacagtcaatgatttaatatcattctcagggattattttatttatattattaacctttggttcaacattaccacttactactctactctcagaaatttctttcaagcattcacctttcaaatatattttgggtttattatcttttccatttatttgaaatgtacttgttctctgtcctttcttttcagactctcgattttcattattctttttgtcagtggtattttttagctttatttgatcactacatttattaactggtctctcctctaatttcttctgctgacttggttttttaccatttgcttcagtccccttgaccggcagcctgtcctcacagtttccagtggactcaccagaaaccaactcacactttaacggctccaagacttcaacatcttgttctcgagttctgaactgttcagaaatgctttcattgctattctgaacaatcatatcttcttcactgctatcctgaatagacacggtatcagaactattttccaaagtgctattagattcagagtcacatcccagttttccttcaaagtccattgctcttgacagaggtgtggcatctctgtcattggtacttttaggcactgatgaatgtaaagcactcttggaagaagaaacaatggtgtcactttcctcctgtatgagcggttttttgttcttacagatcaaagtaccaatatcatctgcactggctagtttagagtcatcgatgaaaaaatcatttccttttgttttactcttactgggttcctggcctctactggcaaggtcagagactttttcttctatgtcattttcaatggaattttgtttcggacattttgtttctgggctccgaatggagacatcatctaacactcgatcttttggataaagtttgtttgtggtatgactaggatcactcattctaagaactgaggaatcactttctgaacatccctgaatcaagtcctcaggttgatcattatttgcatttgggctctgttcttgtctcatcgagtcactctgacacccttcttttgctttcgttattactggtgattcagagagattttttgaagaatttgtagaagtctttcctatacccttaattccaccctccaacttgattttttcgagtcgctgtttttcttccagtgtaaactgtttaattctcctttcaagaagtccatctagtttggatgattttgttttctttttgtaactagtccttagatgaaaaccctcactaacattgaccacatctacttgagaactctcctgacaatttacatgtgactctgttttcatgtcatcgtctacttccattggttcttccttgcagggtttatcactgtcagaatctaagagctccttcacatcttggtccttcttctcagtaatctttgagatatccatttcattttggtctgctccttttgcagcatctgaaccttttacctcatctttttcagaatcaggctctatttttattttttttggacttcgtgaacattttcttttatctgactcatccatattttcatccatattatttttggttccttctaacgactttctgtaattcacattagtattgcctggcaatttaggaacaaacctataaacatgagttttactaatccagctccaaccaccatatcctgtcactctgtactcttcacctttttgtttccaaacctgatgcttaactggaaatgtgtattttacccatgtcgcttgctgcatcgtttcttcttcttcctgtttcttctctttttttttgactttctccttttcttctctttcaattgatgtcatccggtgtaacctggtatgtcctaaagattctcgccatattggtagcatcacaactggtttaactgcacactccaaaatggctaaagccaatgcaaattctctgggtttgctacacatctgaactgccttgatccaatttgccctatgtgatgcccagttgggatgaagaaaggatgaagggatgttgttttctaattgggtgatagtcagtctcagagtagatatggtaagaactttggacccatggacagaaccgttccatttgaactctcctgctggagtcagacagaacttatgtgcaagatgccttctcttatcatggtcttctctgtgctggtgcttattcaaagcaaatgaattggtggagtattgattgtggtagacgcgatacttcccttcttgacccaatttaaaataattgttgatatttcctttcatgatcacttcctttttggtgctcaaccgtgaaatttctccttgagagttaactaccagtacctctttgccctccttaaataatttatttgcttcatgtgcagcggctgccacctgctggctcttcagctgactaagtttgctatctggattccgcaatctggtgatgattcgagttgagccagatgctccttttccagctccaggagattcacttagctccccgttggacttctccgatttgaaatcacctactatctcttcctgaatagagacaggtgtatgagattctctttctccattttcaggatcatcagctgccttagcagattcactctgggaagaatttagttcactgctgctgttactgttttccagattaggctggatggaggtagtggtagcactagtgttactgctctcacatgtcttgttaggttcttctggcacatcctgggggagctcagatgccaccttcttctctgccatgttgctgctatcgggggtttctgagagacaccccacagggctcctcccttcagagggactagtctcttctgaagttgcatttgttgtgttgtcgccaagatttgctgacacagagttacctttatccccaacttctgttggctcctcagattttccttgctcagggtcatcatctggtgttttgtcgtcactgtctttttcaagggactggtcttcaaattcttctctgtttttctcagcatctttagagtcattctcagtctcattcttgtctttttctgtttcttctgggcttttaacattatcaatgtctccctttttggctcttatggattccaaaatttcttcattagctgccgccagaaaggatttgttactgccccgagccttattggtcaggtcttcagttatgtccatgtgtcggtggatttcttcacgcatttcttctagaattttgcagagttctgcttcccaataatctttgtctagacagtcaattaattctgcaagttggacctttgtgctgtaataccaaattttcttttcattttcattttctgtatcttcttctattatgagtcttcggttcaagaaccagtatttcctccgacttctatcatatccaataggttcatgtcgaatatatggtttatttttttggatttcagcaacacagtcagtcacaccaggcaccttgtgtgctacacagacttcacactgccactcgtcctctggcacctcctcaagaggtggcttcacacattccaaatggtatactgctgaacatgtctcacagcaaagcaaatccccaagtttgtgacaaaccctacaatggtcatcatactgtatcaccccttcagacatcaattcctctcgagcaatatttgttgtaagaaactgatcgactagaaactgtagaactttgatcttgttctctactggtccatatgggtagtcctctgcctcttggtaaggaagaacgtgatggtactccttatcactctcacagtacacccgcagcacctctggccacgtcatcccatctatgaaatacagtgtggaattaacgctatctttcagatcagcaggtccaaaggtagtattggaagtgtcttcttcacgcagaactgctttcaaaagcacaacatgcatctctgccatgagtgtgcactgctcttggctcaccagagctgcacaaaagtcctcaaagcgaaaaggagataatctcaaaacagtgccaaagttccgcagtacctcgtaaatggcaatgacattcattatatgctcattaggcaccattaaatcctcagaggacttgggaaattcaaggggcgggatgtctttttcttccaatataggagaacgaggccgatgtactcttggttttcgcctacctggagtgctgctgtaggtactatggctcctgaagctgctttccgtgcagtaactggcgtcgtcgtcgtcgtcttccatctcctccggataatcggagtcatcgtcgtcctcttccatctcatcctcctcgtcgtcctcagaatcctgggtctcctcggcgtcgccgtcctcctcctcctcctcctcggagaccatgtcctcctcttcctcctcctcctcgctctcgtggtcatcgtacaccactttgttgacggccctccgggccgcggtggtccgggccaggtggccgccgccgcccccgccccccgtcctgccgcccccgcctcctcgccccccccggcccggggcgctggtgctggggggggccggcggcggcggcggcggcttcctccggctactgctgccccccctgggcgagctcagccgcgtcttgggcgccacctcagcctgggcggcggcccacctgccccggctgctgccgcggtgccgcgagcggagccccccgatgggtccggacgtgggcggcggcggcggtggcggcggggccggggcgcagcgctccgcagcgggagccgcgggctgcttgggcggcctgccccgccggcccctcatgtcggagccgaggcggggggagaaggaaagcgaagggggaggggcgggcgcagggggggcggtggggagcgccggggccgggtggggaggcccgcggggccgggcgggaggggcccggccgacggaagcgggtggagggagaaggctcaatccgaattgctggggccccactccggatcgccttcagccgccatcttgtttcttccct

SEQ ID NO: 9357 - RNA, 7828 nt, Homo sapiens
  source 1..7828: mol_type = other RNA
aggaagccctggaggggctggaggagctggtgtcactggggggcagggtgcagctactgctgtggcctgagccaactgcatcaggtctttttctttcttaattttcaggtctctcttcagctcttcctgcacttcaatttgcagatccttgtccaggagtgctctcttcttcaggatctcggctctgagctgctctttgtgcttgaagagcagagctgacagcttagtggcattctgcttgctacgtttctgctccacactctcttcacgcttccgtttttttgctgcctgtttttcttctttatctatcttatccaaaatatacttcatcacctggttacagacaatcattctttgattctcttctctttcagctggagtcatgctctttttctgttttaaatgttctattacagcattatgcttcatcaccacctggggttgtgactgtggctggccttgggaaggtatctgaagagatgtatgtggttgaattggaatcggttgtgaggttgtagtctgaacctgggattgttgtccaggagacagttgggatggagttgatggacgtattcgagtctgtgatggactttggacacgaacaggagactgtccttggacattactttgaggctgagactgtgctgcaacttggggcttggatgactgtgcgtgggtgggttgtgcttcagaagggacatgggatgaaacagttgtttgggtctgaacttcaggctgagtctgaacttcaggctgagctggggactggggctgggtttggggctggggctgagctgaaggctgagcagtctgtggctgggcttctgctggacccacacttgatgactgagctggtggcagggttttgtcttgatgtacctgcatctggggtgacagtttactctgcctttgttcacctgtacctgctgctgtcgtggaaacagtggtggtggtggtgctggctgtggtggctgttgttgccaatggggtaaagaggaatcgctgaacagtaccatttggcattgcagcttgcattagctgctggcctgggcctgggagtacagtcaccccttgaggtatcaactgcaactgtccagtagtttgaccttgtccttgaattactactgtcaaaccttgattgccaccgtggccctgtgttaactgagtaagttgagccatggtgagcttcacttgtccttgttgggggcgagggggttgtgaggctgaagactgtatatttgaagtggacgttgctgaagttaagcttttctgcccaggtgttgaggaaaccgtgttaggggcggagactgcagtggagacaggctgccccctgatgatttgagtcatcacttgctgaggagcacctggctgtaccatcacaggtgttcgaataattgcctttcctagtgttgactgttggagtggtgttctaatcacggtcataccagggcgaatctgaggccctgtgattacttgtgaattgcttgtggttcctccagagcctgaggtattgggcctaattgtgactgttgctgtcctgggctggaatgaagtaaaggtttgctgactggtacctgtacttgatggaatgatacccaggactttctgctgtacttgaacaacgcctgaatttgactggccttgcttaacccatgtagcaaaggtttgatgaaagttcttgttttgttggaatgttactgtagctggagatccaactttagtagttagtaccattttggttccagttgtaactgagccacttatgggggccaccataaccttctgtgctggagagatggtgctggttgtactgcttgttggggaagtagtggaagttgcaatcactgtcggcttctgctgctccagtcgtttcttagcctgttgctcaactgcttgtgccttttctttctccactctctcagcaaatgccctgatctcccacaattccagttcttcttctgctacccaggtttcaataataacagggccagtttgcttgggcgtttctggtctctttggccgcagtgcacttgatcgaaggcctttcctctgaggtgtaggcgtttcttttggtgtttctggaactccaatgggacaaatgattttcctgatacaatattcagatcgaatgccataaggaccaacatctctcctcttaattatttctgttgttgtgatttcagtttcggatgtttctgtccgtgtagtccctcctcctggaggagccttggccgccatatcatcccatctcaaacttgcccacagtaaccgtaacatcaggctcactccagctaaggactttactgtctgaagtctatacctccaagtgatgccaaaggtcggtctaggagaaggatatggccatatatccaaagcaggttttgcattgtaattaaaataagggacctctcggattcctccttttcgggccaacttttttaagtcatcattaggcaaaacaaaaatgctcttcttgctgctcttggtaacaaattttctataggatggcagagctgtacctgaacgagtcttctttggtcttgaaaatttcatcagtttcactttgtctcgtgtggaatactctttgctcacagtcatagatgtaaccagtgtgcctcccgtggtggtcagggagtctgtcactgtcgtggtgaccacggttttgctctgctcctttacagagatgatgtccacactgccgcctgtggagggtgtggaaagcttggtcactgttgtagtggtggttgtgacagtggattttgcacaattttctgtggaagaaaccacagtttgcttatcgcctttttctaccttgatcacagtttttgattctgtggccactgtggaggtcatcgtggtgacttctgtgatgacggtttttcttttagattctccattgacattttcatttttgttgatgggcagaccattttcatcaataaagtcattactgagattagattcctcttcagaagtaataggtgatgaagtaactttcttaacttctgaggtttctatttccatatcttctacctgattaactgaattgctttctggacaagatgctgagggtgtggtcgtctgtgtactgtcagactctttggttgatggcagggtctcaaggctatctcggtagttaccttcagcatctgaagaactcagcaaatgcgattttgtttcggagctgtttctttcattaaaatcttccatgatgacatcaccattaatgaatggccttatagcagattctttaacagtcaatgatttaatatcattctcagggattattttatttatattattaacctttggttcaacattaccacttactactctactctcagaaatttctttcaagcattcacctttcaaatatattttgggtttattatcttttccatttatttgaaatgtacttgttctctgtcctttcttttcagactctcgattttcattattctttttgtcagtggtattttttagctttatttgatcactacatttattaactggtctctcctctaatttcttctgctgacttggttttttaccatttgcttcagtccccttgaccggcagcctgtcctcacagtttccagtggactcaccagaaaccaactcacactttaacggctccaagacttcaacatcttgttctcgagttctgaactgttcagaaatgctttcattgctattctgaacaatcatatcttcttcactgctatcctgaatagacacggtatcagaactattttccaaagtgctattagattcagagtcacatcccagttttccttcaaagtccattgctcttgacagaggtgtggcatctctgtcattggtacttttaggcactgatgaatgtaaagcactcttggaagaagaaacaatggtgtcactttcctcctgtatgagcggttttttgttcttacagatcaaagtaccaatatcatctgcactggctagtttagagtcatcgatgaaaaaatcatttccttttgttttactcttactgggttcctggcctctactggcaaggtcagagactttttcttctatgtcattttcaatggaattttgtttcggacattttgtttctgggctccgaatggagacatcatctaacactcgatcttttggataaagtttgtttgtggtatgactaggatcactcattctaagaactgaggaatcactttctgaacatccctgaatcaagtcctcaggttgatcattatttgcatttgggctctgttcttgtctcatcgagtcactctgacacccttcttttgctttcgttattactggtgattcagagagattttttgaagaatttgtagaagtctttcctatacccttaattccaccctccaacttgattttttcgagtcgctgtttttcttccagtgtaaactgtttaattctcctttcaagaagtccatctagtttggatgattttgttttctttttgtaactagtccttagatgaaaaccctcactaacattgaccacatctacttgagaactctcctgacaatttacatgtgactctgttttcatgtcatcgtctacttccattggttcttccttgcagggtttatcactgtcagaatctaagagctccttcacatcttggtccttcttctcagtaatctttgagatatccatttcattttggtctgctccttttgcagcatctgaaccttttacctcatctttttcagaatcaggctctatttttattttttttggacttcgtgaacattttcttttatctgactcatccatattttcatccatattatttttggttccttctaacgactttctgtaattcacattagtattgcctggcaatttaggaacaaacctataaacatgagttttactaatccagctccaaccaccatatcctgtcactctgtactcttcacctttttgtttccaaacctgatgcttaactggaaatgtgtattttacccatgtcgcttgctgcatcgtttcttcttcttcctgtttcttctctttttttttgactttctccttttcttctctttcaattgatgtcatccggtgtaacctggtatgtcctaaagattctcgccatattggtagcatcacaactggtttaactgcacactccaaaatggctaaagccaatgcaaattctctgggtttgctacacatctgaactgccttgatccaatttgccctatgtgatgcccagttgggatgaagaaaggatgaagggatgttgttttctaattgggtgatagtcagtctcagagtagatatggtaagaactttggacccatggacagaaccgttccatttgaactctcctgctggagtcagacagaacttatgtgcaagatgccttctcttatcatggtcttctctgtgctggtgcttattcaaagcaaatgaattggtggagtattgattgtggtagacgcgatacttcccttcttgacccaatttaaaataattgttgatatttcctttcatgatcacttcctttttggtgctcaaccgtgaaatttctccttgagagttaactaccagtacctctttgccctccttaaataatttatttgcttcatgtgcagcggctgccacctgctggctcttcagctgactaagtttgctatctggattccgcaatctggtgatgattcgagttgagccagatgctccttttccagctccaggagattcacttagctccccgttggacttctccgatttgaaatcaccctcagattttccttgctcagggtcatcatctggtgttttgtcgtcactgtctttttcaagggactggtcttcaaattcttctctgtttttctcagcatctttagagtcattctcagtctcattcttgtctttttctgtttcttctgggcttttaacattatcaatgtctccctttttggctcttatggattccaaaatttcttcattagctgccgccagaaaggatttgttactgccccgagccttattggtcaggtcttcagttatgtccatgtgtcggtggatttcttcacgcatttcttctagaattttgcagagttctgcttcccaataatctttgtctagacagtcaattaattctgcaagttggacctttgtgctgtaataccaaattttcttttcattttcattttctgtatcttcttctattatgagtcttcggttcaagaaccagtatttcctccgacttctatcatatccaataggttcatgtcgaatatatggtttatttttttggatttcagcaacacagtcagtcacaccaggcaccttgtgtgctacacagacttcacactgccactcgtcctctggcacctcctcaagaggtggcttcacacattccaaatggtatactgctgaacatgtctcacagcaaagcaaatccccaagtttgtgacaaaccctacaatggtcatcatactgtatcaccccttcagacatcaattcctctcgagcaatatttgttgtaagaaactgatcgactagaaactgtagaactttgatcttgttctctactggtccatatgggtagtcctctgcctcttggtaaggaagaacgtgatggtactccttatcactctcacagtacacccgcagcacctctggccacgtcatcccatctatgaaatacagtgtggaattaacgctatctttcagatcagcaggtccaaaggtagtattggaagtgtcttcttcacgcagaactgctttcaaaagcacaacatgcatctctgccatgagtgtgcactgctcttggctcaccagagctgcacaaaagtcctcaaagcgaaaaggagataatctcaaaacagtgccaaagttccgcagtacctcgtaaatggcaatgacattcattatatgctcattaggcaccattaaatcctcagaggacttgggaaattcaaggggcgggatgtctttttcttccaatataggagaacgaggccgatgtactcttggttttcgcctacctggagtgctgctgtaggtactatggctcctgaagctgctttccgtgcagtaactggcgtcgtcgtcgtcgtcttccatctcctccggataatcggagtcatcgtcgtcctcttccatctcatcctcctcgtcgtcctcagaatcctgggtctcctcggcgtcgccgtcctcctcctcctcctcctcggagaccatgtcctcctcttcctcctcctcctcgctctcgtggtcatcgtacaccactttgttgacggccctccgggccgcggtggtccgggccaggtggccgccgccgcccccgccccccgtcctgccgcccccgcctcctcgccccccccggcccggggcgctggtgctggggggggccggcggcggcggcggcggcttcctccggctactgctgccccccctgggcgagctcagccgcgtcttgggcgccacctcagcctgggcggcggcccacctgccccggctgctgccgcggtgccgcgagcggagccccccgatgggtccggacgtgggcggcggcggcggtggcggcggggccggggcgcagcgctccgcagcgggagccgcgggctgcttgggcggcctgccccgccggcccctcatgtcggagccgaggcggggggagaaggaaagcgaagggggaggggcgggcgcagggggggcggtggggagcgccggggccgggtggggaggcccgcggggccgggcgggaggggcccggccgacggaagcgggtggagggagaaggctcaatccgaattgctggggccccactccggatcgccttcagccgccatcttgtttcttccct

SEQ ID NO: 9358 - RNA, 8209 nt, Homo sapiens
  source 1..8209: mol_type = other RNA
aggaagccctggaggggctggaggagctggtgtcactggggggcagggtgcagctactgctgtggcctgagccaactgcatcaggtctttttctttcttaattttcaggtctctcttcagctcttcctgcacttcaatttgcagatccttgtccaggagtgctctcttcttcaggatctcggctctgagctgctctttgtgcttgaagagcagagctgacagcttagtggcattctgcttgctacgtttctgctccacactctcttcacgcttccgtttttttgctgcctgtttttcttctttatctatcttatccaaaatatacttcatcacctggttacagacaatcattctttgattctcttctctttcagctggagtcatgctctttttctgttttaaatgttctattacagcattatgcttcatcaccacctggggttgtgactgtggctggccttgggaaggtatctgaagagatgtatgtggttgaattggaatcggttgtgaggttgtagtctgaacctgggattgttgtccaggagacagttgggatggagttgatggacgtattcgagtctgtgatggactttggacacgaacaggagactgtccttggacattactttgaggctgagactgtgctgcaacttggggcttggatgactgtgcgtgggtgggttgtgcttcagaagggacatgggatgaaacagttgtttgggtctgaacttcaggctgagtctgaacttcaggctgagctggggactggggctgggtttggggctggggctgagctgaaggctgagcagtctgtggctgggcttctgctggacccacacttgatgactgagctggtggcagggttttgtcttgatgtacctgcatctggggtgacagtttactctgcctttgttcacctgtacctgctgctgtcgtggaaacagtggtggtggtggtgctggctgtggtggctgttgttgccaatggggtaaagaggaatcgctgaacagtaccatttggcattgcagcttgcattagctgctggcctgggcctgggagtacagtcaccccttgaggtatcaactgcaactgtccagtagtttgaccttgtccttgaattactactgtcaaaccttgattgccaccgtggccctgtgttaactgagtaagttgagccatggtgagcttcacttgtccttgttgggggcgagggggttgtgaggctgaagactgtatatttgaagtggacgttgctgaagttaagcttttctgcccaggtgttgaggaaaccgtgttaggggcggagactgcagtggagacaggctgccccctgatgatttgagtcatcacttgctgaggagcacctggctgtaccatcacaggtgttcgaataattgcctttcctagtgttgactgttggagtggtgttctaatcacggtcataccagggcgaatctgaggccctgtgattacttgtgaattgcttgtggttcctccagagcctgaggtattgggcctaattgtgactgttgctgtcctgggctggaatgaagtaaaggtttgctgactggtacctgtacttgatggaatgatacccaggactttctgctgtacttgaacaacgcctgaatttgactggccttgcttaacccatgtagcaaaggtttgatgaaagttcttgttttgttggaatgttactgtagctggagatccaactttagtagttagtaccattttggttccagttgtaactgagccacttatgggggccaccataaccttctgtgctggagagatggtgctggttgtactgcttgttggggaagtagtggaagttgcaatcactgtcggcttctgctgctccagtcgtttcttagcctgttgctcaactgcttgtgccttttctttctccactctctcagcaaatgccctgatctcccacaattccagttcttcttctgctacccaggtttcaataataacagggccagtttgcttgggcgtttctggtctctttggccgcagtgcacttgatcgaaggcctttcctctgaggtgtaggcgtttcttttggtgtttctggaactccaatgggacaaatgattttcctgatacaatattcagatcgaatgccataaggaccaacatctctcctcttaattatttctgttgttgtgatttcagtttcggatgtttctgtccgtgtagtccctcctcctggaggagccttggccgccatatcatcccatctcaaacttgcccacagtaaccgtaacatcaggctcactccagctaaggactttactgtctgaagtctatacctccaagtgatgccaaaggtcggtctaggagaaggatatggccatatatccaaagcaggttttgcattgtaattaaaataagggacctctcggattcctccttttcgggccaacttttttaagtcatcattaggcaaaacaaaaatgctcttcttgctgctcttggtaacaaattttctataggatggcagagctgtacctgaacgagtcttctttggtcttgaaaatttcatcagtttcactttgtctcgtgtggaatactctttgctcacagtcatagatgtaaccagtgtgcctcccgtggtggtcagggagtctgtcactgtcgtggtgaccacggttttgctctgctcctttacagagatgatgtccacactgccgcctgtggagggtgtggaaagcttggtcactgttgtagtggtggttgtgacagtggattttgcacaattttctgtggaagaaaccacagtttgcttatcgcctttttctaccttgatcacagtttttgattctgtggccactgtggaggtcatcgtggtgacttctgtgatgacggtttttcttttagattctccattgacattttcatttttgttgatgggcagaccattttcatcaataaagtcattactgagattagattcctcttcagaagtaataggtgatgaagtaactttcttaacttctgaggtttctatttccatatcttctacctgattaactgaattgctttctggacaagatgctgagggtgtggtcgtctgtgtactgtcagactctttggttgatggcagggtctcaaggctatctcggtagttaccttcagcatctgaagaactcagcaaatgcgattttgtttcggagctgtttctttcattaaaatcttccatgatgacatcaccattaatgaatggccttatagcagattctttaacagtcaatgatttaatatcattctcagggattattttatttatattattaacctttggttcaacattaccacttactactctactctcagaaatttctttcaagcattcacctttcaaatatattttgggtttattatcttttccatttatttgaaatgtacttgttctctgtcctttcttttcagactctcgattttcattattctttttgtcagtggtattttttagctttatttgatcactacatttattaactggtctctcctctaatttcttctgctgacttggttttttaccatttgcttcagtccccttgaccggcagcctgtcctcacagtttccagtggactcaccagaaaccaactcacactttaacggctccaagacttcaacatcttgttctcgagttctgaactgttcagaaatgctttcattgctattctgaacaatcatatcttcttcactgctatcctgaatagacacggtatcagaactattttccaaagtgctattagattcagagtcacatcccagttttccttcaaagtccattgctcttgacagaggtgtggcatctctgtcattggtacttttaggcactgatgaatgtaaagcactcttggaagaagaaacaatggtgtcactttcctcctgtatgagcggttttttgttcttacagatcaaagtaccaatatcatctgcactggctagtttagagtcatcgatgaaaaaatcatttccttttgttttactcttactgggttcctggcctctactggcaaggtcagagactttttcttctatgtcattttcaatggaattttgtttcggacattttgtttctgggctccgaatggagacatcatctaacactcgatcttttggataaagtttgtttgtggtatgactaggatcactcattctaagaactgaggaatcactttctgaacatccctgaatcaagtcctcaggttgatcattatttgcatttgggctctgttcttgtctcatcgagtcactctgacacccttcttttgctttcgttattactggtgattcagagagattttttgaagaatttgtagaagtctttcctatacccttaattccaccctccaacttgattttttcgagtcgctgtttttcttccagtgtaaactgtttaattctcctttcaagaagtccatctagtttggatgattttgttttctttttgtaactagtccttagatgaaaaccctcactaacattgaccacatctacttgagaactctcctgacaatttacatgtgactctgttttcatgtcatcgtctacttccattggttcttccttgcagggtttatcactgtcagaatctaagagctccttcacatcttggtccttcttctcagtaatctttgagatatccatttcattttggtctgctccttttgcagcatctgaaccttttacctcatctttttcagaatcaggctctatttttattttttttggacttcgtgaacattttcttttatctgactcatccatattttcatccatattatttttggttccttctaacgactttctgtaattcacattagtattgcctggcaatttaggaacaaacctataaacatgagttttactaatccagctccaaccaccatatcctgtcactctgtactcttcacctttttgtttccaaacctgatgcttaactggaaatgtgtattttacccatgtcgcttgctgcatcgtttcttcttcttcctgtttcttctctttttttttgactttctccttttcttctctttcaattgatgtcatccggtgtaacctggtatgtcctaaagattctcgccatattggtagcatcacaactggtttaactgcacactccaaaatggctaaagccaatgcaaattctctgggtttgctacacatctgaactgccttgatccaatttgccctatgtgatgcccagttgggatgaagaaaggatgaagggatgttgttttctaattgggtgatagtcagtctcagagtagatatggtaagaactttggacccatggacagaaccgttccatttgaactctcctgctggagtcagacagaacttatgtgcaagatgccttctcttatcatggtcttctctgtgctggtgcttattcaaagcaaatgaattggtggagtattgattgtggtagacgcgatacttcccttcttgacccaatttaaaataattgttgatatttcctttcatgatcacttcctttttggtgctcaaccgtgaaatttctccttgagagttaactaccagtacctctttgccctccttaaataatttatttgcttcatgtgcagcggctgccacctgctggctcttcagctgactaagtttgctatctggattccgcaatctggtgatgattcgagttgagccagatgctccttttccagctccaggagattcacttagctccccgttggacttctccgatttgaaatcacctactatctcttcctgaatagagacaggtgtatgagattctctttctccattttcaggatcatcagctgccttagcagattcactctgggaagaatttagttcactgctgctgttactgttttccagattaggctggatggaggtagtggtagcactagtgttactgctctcacatgtcttgttaggttcttctggcacatcctgggggagctcagatgccaccttcttctctgccatgttgctgctatcgggggtttctgagagacaccccacagggctcctcccttcagagggactagtctcttctgaagttgcatttgttgtgttgtcgccaagatttgctgacacagagttacctttatccccaacttctgttggctcctcagattttccttgctcagggtcatcatctggtgttttgtcgtcactgtctttttcaagggactggtcttcaaattcttctctgtttttctcagcatctttagagtcattctcagtctcattcttgtctttttctgtttcttctgggcttttaacattatcaatgtctccctttttggctcttatggattccaaaatttcttcattagctgccgccagaaaggatttgttactgccccgagccttattggtcaggtcttcagttatgtccatgtgtcggtggatttcttcacgcatttcttctagaattttgcagagttctgcttcccaataatctttgtctagacagtcaattaattctgcaagttggacctttgtgctgtaataccaaattttcttttcattttcattttctgtatcttcttctattatgagtcttcggttcaagaaccagtatttcctccgacttctatcatatccaataggttcatgtcgaatatatggtttatttttttggatttcagcaacacagtcagtcacaccaggcaccttgtgtgctacacagacttcacactgccactcgtcctctggcacctcctcaagaggtggcttcacacattccaaatggtatactgctgaacatgtctcacagcaaagcaaatccccaagtttgtgacaaaccctacaatggtcatcatactgtatcaccccttcagacatcaattcctctcgagcaatatttgttgtaagaaactgatcgactagaaactgtagaactttgatcttgttctctactggtccatatgggtagtcctctgcctcttggtaaggaagaacgtgatggtactccttatcactctcacagtacacccgcagcacctctggccacgtcatcccatctatgaaatacagtgtggaattaacgctatctttcagatcagcaggtccaaaggtagtattggaagtgtcttcttcacgcagaactgctttcaaaagcacaacatgcatctctgccatgagtgtgcactgctcttggctcaccagagctgcacaaaagtcctcaaagcgaaaaggagataatctcaaaacagtgccaaagttccgcagtacctcgtaaatggcaatgacattcattatatgctcattaggcaccattaaatcctcagaggacttgggaaattcaaggggcgggatgtctttttcttccaatataggagaacgaggccgatgtactcttggttttcgcctacctggagtgctgctgtaggtactatggctcctgaagctgctttccgtgcagtaactggcgtcgtcgtcgtcgtcttccatctcctccggataatcggagtcatcgtcgtcctcttccatctcatcctcctcgtcgtcctcagaatcctgggtctcctcggcgtcgccgtcctcctcctcctcctcctcggagaccatgtcctcctcttcctcctcctcctcgctctcgtggtcatcgtacaccactttgttgacggccctccgggccgcggtggtccgggccaggtggccgccgccgcccccgccccccgtcctgccgcccccgcctcctcgccccccccggcccggggcgctggtgctggggggggccggcggcggcggcggcggcttcctccggctactgctgccccccctgggcgagctcagccgcgtcttgggcgccacctcagcctgggcggcggcccacctgccccggctgctgccgcggtgccgcgagcggagccccccgatgggtccggacgtgggcggcggcggcggtggcggcggggccggggcgcagcgctccgcagcgggagccgcgggctgcttgggcggcctgccccgccggcccctcatgtcggagccgaggcggggggagaaggaaagcgaagggggaggggcgggcgcagggggggcggtggggagcgccggggccgggtggggaggcccgcggggccgggcgggaggggcccggccgacggaagcgggtggagggagaaggctcaatccgaattgctggggccccactccggatcgccttcagccgccatcttgtttcttccct

SEQ ID NO: 9359 - RNA, 8223 nt, Homo sapiens
  source 1..8223: mol_type = other RNA
aggaagccctggaggggctggaggagctggtgtcactggggggcagggtgcagctactgctgtggcctgagccaactgcatcaggtctttttctttcttaattttcaggtctctcttcagctcttcctgcacttcaatttgcagatccttgtccaggagtgctctcttcttcaggatctcggctctgagctgctctttgtgcttgaagagcagagctgacagcttagtggcattctgcttgctacgtttctgctccacactctcttcacgcttccgtttttttgctgcctgtttttcttctttatctatcttatccaaaatatacttcatcacctggttacagacaatcattctttgattctcttctctttcagctggagtcatgctctttttctgttttaaatgttctattacagcattatgcttcatcaccacctggggttgtgactgtggctggccttgggaaggtatctgaagagatgtatgtggttgaattggaatcggttgtgaggttgtagtctgaacctgggattgttgtccaggagacagttgggatggagttgatggacgtattcgagtctgtgatggactttggacacgaacaggagactgtccttggacattactttgaggctgagactgtgctgcaacttggggcttggatgactgtgcgtgggtgggttgtgcttcagaagggacatgggatgaaacagttgtttgggtctgaacttcaggctgagtctgaacttcaggctgagctggggactggggctgggtttggggctggggctgagctgaaggctgagcagtctgtggctgggcttctgctggacccacacttgatgactgagctggtggcagggttttgtcttgatgtacctgcatctggggtgacagtttactctgcctttgttcacctgtacctgctgctgtcgtggaaacagtggtggtggtggtgctggctgtggtggctgttgttgccaatggggtaaagaggaatcgctgaacagtaccatttggcattgcagcttgcattagctgctggcctgggcctgggagtacagtcaccccttgaggtatcaactgcaactgtccagtagtttgaccttgtccttgaattactactgtcaaaccttgattgccaccgtggccctgtgttaactgagtaagttgagccatggtgagcttcacttgtccttgttgggggcgagggggttgtgaggctgaagactgtatatttgaagtggacgttgctgaagttaagcttttctgcccaggtgttgaggaaaccgtgttaggggcggagactgcagtggagacaggctgccccctgatgatttgagtcatcacttgctgaggagcacctggctgtaccatcacaggtgttcgaataattgcctttcctagtgttgactgttggagtggtgttctaatcacggtcataccagggcgaatctgaggccctgtgattacttgtgaattgcttgtggttcctccagagcctgaggtattgggcctaattgtgactgttgctgtcctgggctggaatgaagtaaaggtttgctgactggtacctgtacttgatggaatgatacccaggactttctgctgtacttgaacaacgcctgaatttgactggccttgcttaacccatgtagcaaaggtttgatgaaagttcttgttttgttggaatgttactgtagctggagatccaactttagtagttagtaccattttggttccagttgtaactgagccacttatgggggccaccataaccttctgtgctggagagatggtgctggttgtactgcttgttggggaagtagtggaagttgcaatcactgtcggcttctgctgctccagtcgtttcttagcctgttgctcaactgcttgtgccttttctttctccactctctcagcaaatgccctgatctcccacaattccagttcttcttctgctacccaggtttcaataataacagggccagtttgcttgggcgtttctggtctctttggccgcagtgcacttgatcgaaggcctttcctctgaggtgtaggcgtttcttttggtgtttctggaactccaatgggacaaatgattttcctgatacaatattcagatcgaatgccataaggaccaacatctctcctcttaattatttctgttgttgtgatttcagtttcggatgtttctgtccgtgtagtccctcctcctggaggagccttggccgccatatcatcccatctcaaacttgcccacagtaaccgtaacatcaggctcactccagctaaggactttactgtctgaagtctatacctccaagtgatgccaaaggtcggtctaggagaaggatatggccatatatccaaagcaggttttgcattgtaattaaaataagggacctctcggattcctccttttcgggccaacttttttaagtcatcattaggcaaaacaaaaatgctcttcttgctgctcttggtaacaaattttctataggatggcagagctgtacctgaacgagtcttctttggtcttgaaaatttcatcagtttcactttgtctcgtgtggaatactctttgctcacagtcatagatgtaaccagtgtgcctcccgtggtggtcagggagtctgtcactgtcgtggtgaccacggttttgctctgctcctttacagagatgatgtccacactgccgcctgtggagggtgtggaaagcttggtcactgttgtagtggtggttgtgacagtggattttgcacaattttctgtggaagaaaccacagtttgcttatcgcctttttctaccttgatcacagtttttgattctgtggccactgtggaggtcatcgtggtgacttctgtgatgacggtttttcttttagattctccattgacattttcatttttgttgatgggcagaccattttcatcaataaagtcattactgagattagattcctcttcagaagtaataggtgatgaagtaactttcttaacttctgaggtttctatttccatatcttctacctgattaactgaattgctttctggacaagatgctgagggtgtggtcgtctgtgtactgtcagactctttggttgatggcagggtctcaaggctatctcggtagttaccttcagcatctgaagaactcagcaaatgcgattttgtttcggagctgtttctttcattaaaatcttccatgatgacatcaccattaatgaatggccttatagcagattctttaacagtcaatgatttaatatcattctcagggattattttatttatattattaacctttggttcaacattaccacttactactctactctcagaaatttctttcaagcattcacctttcaaatatattttgggtttattatcttttccatttatttgaaatgtacttgttctctgtcctttcttttcagactctcgattttcattattctttttgtcagtggtattttttagctttatttgatcactacatttattaactggtctctcctctaatttcttctgctgacttggttttttaccatttgcttcagtccccttgaccggcagcctgtcctcacagtttccagtggactcaccagaaaccaactcacactttaacggctccaagacttcaacatcttgttctcgagttctgaactgttcagaaatgctttcattgctattctgaacaatcatatcttcttcactgctatcctgaatagacacggtatcagaactattttccaaagtgctattagattcagagtcacatcccagttttccttcaaagtccattgctcttgacagaggtgtggcatctctgtcattggtacttttaggcactgatgaatgtaaagcactcttggaagaagaaacaatggtgtcactttcctcctgtatgagcggttttttgttcttacagatcaaagtaccaatatcatctgcactggctagtttagagtcatcgatgaaaaaatcatttccttttgttttactcttactgggttcctggcctctactggcaaggtcagagactttttcttctatgtcattttcaatggaattttgtttcggacattttgtttctgggctccgaatggagacatcatctaacactcgatcttttggataaagtttgtttgtggtatgactaggatcactcattctaagaactgaggaatcactttctgaacatccctgaatcaagtcctcaggttgatcattatttgcatttgggctctgttcttgtctcatcgagtcactctgacacccttcttttgctttcgttattactggtgattcagagagattttttgaagaatttgtagaagtctttcctatacccttaattccaccctccaacttgattttttcgagtcgctgtttttcttccagtgtaaactgtttaattctcctttcaagaagtccatctagtttggatgattttgttttctttttgtaactagtccttagatgaaaaccctcactaacattgaccacatctacttgagaactctcctgacaatttacatgtgactctgttttcatgtcatcgtctacttccattggttcttccttgcagggtttatcactgtcagaatctaagagctccttcacatcttggtccttcttctcagtaatctttgagatatccatttcattttggtctgctccttttgcagcatctgaaccttttacctcatctttttcagaatcaggctctatttttattttttttggacttcgtgaacattttcttttatctgactcatccatattttcatccatattatttttggttccttctaacgactttctgtaattcacattagtattgcctggcaatttaggaacaaacctataaacatgagttttactaatccagctccaaccaccatatcctgtcactctgtactcttcacctttttgtttccaaacctgatgcttaactggaaatgtgtattttacccatgtcgcttgctgcatcgtttcttcttcttcctgtttcttctctttttttttgactttctccttttcttctctttcaattgatgtcatccggtgtaacctggtatgtcctaaagattctcgccatattggtagcatcacaactggtttaactgcacactccaaaatggctaaagccaatgcaaattctctgggtttgctacacatctgaactgccttgatccaatttgccctatgtgatgcccagttgggatgaagaaaggatgaagggatgttgttttctaattgggtgatagtcagtctcagagtagatatggtaagaactttggacccatggacagaaccgttccatttgaactctcctgctggagtcagacagaacttatgtgcaagatgccttctcttatcatggtcttctctgtgctggtgcttattcaaagcaaatgaattggtggagtattgattgtggtagacgcgatacttcccttcttgacccaatttaaaataattgttgatatttcctttcatgatcacttcctttttggtgctcaaccgtgaaatttctccttgagagttaactaccagtacctctttgccctccttaaataatttatttgcttcatgtgcagcggctgccacctgctggctcttcagctgactaagtttgctatctggattccgcaatctggtgatgattcgagttgagccagatgctccttttccagctccaggagattcacttagctccccgttggacttctccgatttgaaatcacctactatctcttcctgaatagagacaggtgtatgagattctctttctccattttcaggatcatcagctgccttagcagattcactctgggaagaatttagttcactgctgctgttactgttttccagattaggctggatggaggtagtggtagcactagtgttactgctctcacatgtcttgttaggttcttctggcacatcctgggggagctcagatgccaccttcttctctgccatgttgctgctatcgggggtttctgagagacaccccacagggctcctcccttcagagggactagtctcttctgaagttgcatttgttgtgttgtcgccaagatttgctgacacagagttacctttatccccaacttctgttggctcctcagattttccttgctcagggtcatcatctggtgttttgtcgtcactgtctttttcaagggactggtcttcaaattcttctctgtttttctcagcatctttagagtcattctcagtctcattcttgtctttttctgtttcttctgggcttttaacattatcaatgtctccctttttggctcttatggattccaaaatttcttcattagctgccgccagaaaggatttgttactgccccgagccttattggtcaggtcttcagttatgtccatgtgtcggtggatttcttcacgcatttcttctagaattttgcagagttctgcttcccaataatctttgtctagacagtcaattaattctgcaagttggacctttgtgctgtaataccaaattttcttttcattttcattttctgtatcttcttctattatgagtcttcggttcaagaaccagtatttcctccgacttctatcatatccaataggttcatgtcgaatatatggtttatttttttggatttcagcaacacagtcagtcacaccaggcaccttgtgtgctacacagacttcacactgccactcgtcctctggcacctcctcaagaggtggcttcacacattccaaatggtatactgctgaacatgtctcacagcaaagcaaatccccaagtttgtgacaaaccctacaatggtcatcatactgtatcaccccttcagacatcaattcctctcgagcaatatttgttgtaagaaactgatcgactagaaactgtagaactttgatcttgttctctactggtccatatgggtagtcctctgcctcttggtaaggaagaacgtgatggtactccttatcactctcacagtacacccgcagcacctctggccacgtcatcccatctatgaaatacagtgtggaattaacgctatctttcagatcagcaggtccaaaggtagtattggaagtgtcttcttcacgcagaactgctttcaaaagcacaacatgcatctctgccatgagtgtgcactgctcttggctcaccagagctgcacaaaagtcctcaaagcgaaaaggagataatctcaaaacagtgccaaagttccgcagtacctcgtaaatggcaatgacattcattatatgctcattaggcaccattaaatcctcagaggacttgggaaattcaaggggcgggatgtctttttcttccaatataggagaacgaggccgatgtactcttggttttcgcctacctggagtgctgctgtaggtactatggctcctgaagctgctttccgtgcagtaactggcgtcgtcgtcgtcgtcttccatctcctccggataatcggagtcatcgtcgtcctcttccatctcatcctcctcgtcgtcctcagaatcctgggtctcctcggcgtcgccgtcctcctcctcctcctcctcggagaccatgtcctcctcttcctcctcctcctcgctctcgtggtcatcgtacaccactttgttgacggccctccgggccgcggtggtccgggccaggtggccgccgccgcccccgccccccgtcctgccgcccccgcctcctcgccccccccggcccggggcgctggtgctggggggggccggcggcggcggcggcggcttcctccggctactgctgccccccctgggcgagctcagccgcgtcttgggcgccacctcagcctgggcggcggcccacctgccccggctgctgccgcggtgccgcgagcggagccccccgatgggtccggacgtgggcggcggcggcggtggcggcggggccggggcgcagcgctccgcagcgggagccgcgggctgcttgggcggcctgccccgccggcccctcatgtcggagccgaggcggggggagaaggaaagcgaagggggaggggcgggcgcagggggggcggtggggagcgccggggccgggtggggaggcccgcggggccgggcgggaggggcccggccgacggaagcgggtggagggagaaggctcaatccgaattgctggggccccactccggatcgccttcagccgccatcttgtttcttccctctcgctcggtgact

SEQ ID NO: 9360 - RNA, 6366 nt, Homo sapiens
  source 1..6366: mol_type = other RNA
aggaagccctggaggggctggaggagctggtgtcactggggggcagggtgcagctactgctgtggcctgagccaactgcatcaggtctttttctttcttaattttcaggtctctcttcagctcttcctgcacttcaatttgcagatccttgtccaggagtgctctcttcttcaggatctcggctctgagctgctctttgtgcttgaagagcagagctgacagcttagtggcattctgcttgctacgtttctgctccacactctcttcacgcttccgtttttttgctgcctgtttttcttctttatctatcttatccaaaatatacttcatcacctggttacagacaatcattctttgattctcttctctttcagctggagtcatgctctttttctgttttaaatgttctattacagcattatgcttcatcaccacctgtttctgaatgatttcactttgattagaagcttggagggtgtgttcacgcttaatttctatctgttgctgtttcttcttttgctgctgatccctgagttgctgaaccctttgcaactgctcttgcacactggctgcctgcactgtaaccacattctgaatctggtgagtctgcacagcactgctttgctgaatttggataggtaactggagtttgatttgctggggcacaccactttgctgagcctgtatctgagccacaacctgtgactggatctgagagagaacctggacttgttgttgcagctgaggcacagcaatgacttggggctgtggctgctgtatttgtagctgaggacgggatggggatgaaacagtaacttgatttaaagtttgtcctgatgaaagagtttgagttgaagactgtacctggggttgtgactgtggctggccttgggaaggtatctgaagagatgtatgtggttgaattggaatcggttgtgaggttgtagtctgaacctgggattgttgtccaggagacagttgggatggagttgatggacgtattcgagtctgtgatggactttggacacgaacaggagactgtccttggacattactttgaggctgagactgtgctgcaacttggggcttggatgactgtgcgtgggtgggttgtgcttcagaagggacatgggatgaaacagttgtttgggtctgaacttcaggctgagtctgaacttcaggctgagctggggactggggctgggtttggggctggggctgagctgaaggctgagcagtctgtggctgggcttctgctggacccacacttgatgactgagctggtggcagggttttgtcttgatgtacctgcatctggggtgacagtttactctgcctttgttcacctgtacctgctgctgtcgtggaaacagtggtggtggtggtgctggctgtggtggctgttgttgccaatggggtaaagaggaatcgctgaacagtaccatttggcattgcagcttgcattagctgctggcctgggcctgggagtacagtcaccccttgaggtatcaactgcaactgtccagtagtttgaccttgtccttgaattactactgtcaaaccttgattgccaccgtggccctgtgttaactgagtaagttgagccatggtgagcttcacttgtccttgttgggggcgagggggttgtgaggctgaagactgtatatttgaagtggacgttgctgaagttaagcttttctgcccaggtgttgaggaaaccgtgttaggggcggagactgcagtggagacaggctgccccctgatgatttgagtcatcacttgctgaggagcacctggctgtaccatcacaggtgttcgaataattgcctttcctagtgttgactgttggagtggtgttctaatcacggtcataccagggcgaatctgaggccctgtgattacttgtgaattgcttgtggttcctccagagcctgaggtattgggcctaattgtgactgttgctgtcctgggctggaatgaagtaaaggtttgctgactggtacctgtacttgatggaatgatacccaggactttctgctgtacttgaacaacgcctccttgtgttgctggcacatttacagcgacaatcttgctgtttgcaggaagtggcagtttggtaattacttttcctgccatagtgactggattgcctgtaatttggaacgtctgacctgtgctggcaatggttgtagcagatgtggcagctgtgctggtggctgaatttgactggccttgcttaacccatgtagcaaaggtttgatgaaagttcttgttttgttggaatgttactgtagctggagatccaactttagtagttagtaccattttggttccagttgtaactgagccacttatgggggccaccataaccttctgtgctggagagatggtgctggttgtactgcttgttggggaagtagtggaagttgcaatcactgtcggcttctgctgctccagtcgtttcttagcctgttgctcaactgcttgtgccttttctttctccactctctcagcaaatgccctgatctcccacaattccagttcttcttctgctacccaggtttcaataataacagggccagtttgcttgggcgtttctggtctctttggccgcagtgcacttgatcgaaggcctttcctctgaggtgtaggcgtttcttttggtgtttctggaactccaatgggacaaatgattttcctgatacaatattcagatcgaatgccataaggaccaacatctctcctcttaattatttctgttgttgtgatttcagtttcggatgtttctgtccgtgtagtccctcctcctggaggagccttggccgccatatcatcccatctcaaacttgcccacagtaaccgtaacatcaggctcactccagctaaggactttactgtctgaagtctatacctccaagtgatgccaaaggtcggtctaggagaaggatatggccatatatccaaagcaggttttgcattgtaattaaaataagggacctctcggattcctccttttcgggccaacttttttaagtcatcattaggcaaaacaaaaatgctcttcttgctgctcttggtaacaaattttctataggatggcagagctgtacctgaacgagtcttctttggtcttgaaaatttcatcagtttcactttgtctcgtgtggaatactctttgctcacagtcatagatgtaaccagtgtgcctcccgtggtggtcagggagtctgtcactgtcgtggtgaccacggttttgctctgctcctttacagagatgatgtccacactgccgcctgtggagggtgtggaaagcttggtcactgttgtagtggtggttgtgacagtggattttgcacaattttctgtggaagaaaccacagtttgcttatcgcctttttctaccttgatcacagtttttgattctgtggccactgtggaggtcatcgtggtgacttctgtgatgacggtttttcttttagattctccattgacattttcatttttgttgatgggcagaccattttcatcaataaagtcattactgagattagattcctcttcagaagtaataggtgatgaagtaactttcttaacttctgaggtttctatttccatatcttctacctgattaactgaattgctttctggacaagatgctgagggtgtggtcgtctgtgtactgtcagactctttggttgatggcagggtctcaaggctatctcggtagttaccttcagcatctgaagaactcagcaaatgcgattttgtttcggagctgtttctttcattaaaatcttccatgatgacatcaccattaatgaatggccttatagcagattctttaacagtcaatgatttaatatcattctcagggattattttatttatattattaacctttggttcaacattaccacttactactctactctcagaaatttctttcaagcattcacctttcaaatatattttgggtttattatcttttccatttatttgaaatgtacttgttctctgtcctttcttttcagactctcgattttcattattctttttgtcagtggtattttttagctttatttgatcactacatttattaactggtctctcctctaatttcttctgctgacttggttttttaccatttgcttcagtccccttgaccggcagcctgtcctcacagtttccagtggactcaccagaaaccaactcacactttaacggctccaagacttcaacatcttgttctcgagttctgaactgttcagaaatgctttcattgctattctgaacaatcatatcttcttcactgctatcctgaatagacacggtatcagaactattttccaaagtgctattagattcagagtcacatcccagttttccttcaaagtccattgctcttgacagaggtgtggcatctctgtcattggtacttttaggcactgatgaatgtaaagcactcttggaagaagaaacaatggtgtcactttcctcctgtatgagcggttttttgttcttacagatcaaagtaccaatatcatctgcactggctagtttagagtcatcgatgaaaaaatcatttccttttgttttactcttactgggttcctggcctctactggcaaggtcagagactttttcttctatgtcattttcaatggaattttgtttcggacattttgtttctgggctccgaatggagacatcatctaacactcgatcttttggataaagtttgtttgtggtatgactaggatcactcattctaagaactgaggaatcactttctgaacatccctgaatcaagtcctcaggttgatcattatttgcatttgggctctgttcttgtctcatcgagtcactctgacacccttcttttgctttcgttattactggtgattcagagagattttttgaagaatttgtagaagtctttcctatacccttaattccaccctccaacttgattttttcgagtcgctgtttttcttccagtgtaaactgtttaattctcctttcaagaagtccatctagtttggatgattttgttttctttttgtaactagtccttagatgaaaaccctcactaacattgaccacatctacttgagaactctcctgacaatttacatgtgactctgttttcatgtcatcgtctacttccattggttcttccttgcagggtttatcactgtcagaatctaagagctccttcacatcttggtccttcttctcagtaatctttgagatatccatttcattttggtctgctccttttgcagcatctgaaccttttacctcatctttttcagaatcaggctctatttttattttttttggacttcgtgaacattttcttttatctgactcatccatattttcatccatattatttttggttccttctaacgactttctgtaattcacattagtattgcctggcaatttaggaacaaacctataaacatgagttttactaatccagctccaaccaccatatcctgtcactctgtactcttcacctttttgtttccaaacctgatgcttaactggaaatgtgtattttacccatgtcgcttgctgcatcgtttcttcttcttcctgtttcttctctttttttttgactttctccttttcttctctttcaattgatgtcatccggtgtaacctggtatgtcctaaagattctcgccatattggtagcatcacaactggtttaactgcacactccaaaatggctaaagccaatgcaaattctctgggtttgctacacatctgaactgccttgatccaatttgccctatgtgatgcccagttgggatgaagaaaggatgaagggatgttgttttctaattgggtgatagtcagtctcagagtagatatggtaagaactttggacccatggacagaaccgttccatttgaactctcctgctggagtcagacagaacttatgtgcaagatgccttctcttatcatggtcttctctgtgctggtgcttattcaaagcaaatgaattggtggagtattgattgtggtagacgcgatacttcccttcttgacccaatttaaaataattgttgatatttcctttcatgatcacttcctttttggtgctcaaccgtgaaatttctccttgagagttaactaccagtacctctttgccctccttaaataataagtcaaaatggagagagggtactgagcatcttgccaccccaggctggaaagcaagtcactttggatgtgtggtagcaaagcagttggtcagactatcaattttctcttgggtctcagatcatggaggttttttttcttttttttgagatggagtttcgctcttgtcgcccaggctggagtgcag

SEQ ID NO: 9361 - RNA, 8419 nt, Homo sapiens
  source 1..8419: mol_type = other RNA
aggaagccctggaggggctggaggagctggtgtcactggggggcagggtgcagctactgctgtggcctgagccaactgcatcaggtctttttctttcttaattttcaggtctctcttcagctcttcctgcacttcaatttgcagatccttgtccaggagtgctctcttcttcaggatctcggctctgagctgctctttgtgcttgaagagcagagctgacagcttagtggcattctgcttgctacgtttctgctccacactctcttcacgcttccgtttttttgctgcctgtttttcttctttatctatcttatccaaaatatacttcatcacctggttacagacaatcattctttgattctcttctctttcagctggagtcatgctctttttctgttttaaatgttctattacagcattatgcttcatcaccacctgtttctgaatgatttcactttgattagaagcttggagggtgtgttcacgcttaatttctatctgttgctgtttcttcttttgctgctgatccctgagttgctgaaccctttgcaactgctcttgcacactggctgcctgcactgtaaccacattctgaatctggtgagtctgcacagcactgctttgctgaatttggataggtaactggagtttgatttgctggggcacaccactttgctgagcctgtatctgagccacaacctgtgactggatctgagagagaacctggacttgttgttgcagctgaggcacagcaatgacttggggctgtggctgctgtatttgtagctgaggacgggatggggatgaaacagtaacttgatttaaagtttgtcctgatgaaagagtttgagttgaagactgtacctggggttgtgactgtggctggccttgggaaggtatctgaagagatgtatgtggttgaattggaatcggttgtgaggttgtagtctgaacctgggattgttgtccaggagacagttgggatggagttgatggacgtattcgagtctgtgatggactttggacacgaacaggagactgtccttggacattactttgaggctgagactgtgctgcaacttggggcttggatgactgtgcgtgggtgggttgtgcttcagaagggacatgggatgaaacagttgtttgggtctgaacttcaggctgagtctgaacttcaggctgagctggggactggggctgggtttggggctggggctgagctgaaggctgagcagtctgtggctgggcttctgctggacccacacttgatgactgagctggtggcagggttttgtcttgatgtacctgcatctggggtgacagtttactctgcctttgttcacctgtacctgctgctgtcgtggaaacagtggtggtggtggtgctggctgtggtggctgttgttgccaatggggtaaagaggaatcgctgaacagtaccatttggcattgcagcttgcattagctgctggcctgggcctgggagtacagtcaccccttgaggtatcaactgcaactgtccagtagtttgaccttgtccttgaattactactgtcaaaccttgattgccaccgtggccctgtgttaactgagtaagttgagccatggtgagcttcacttgtccttgttgggggcgagggggttgtgaggctgaagactgtatatttgaagtggacgttgctgaagttaagcttttctgcccaggtgttgaggaaaccgtgttaggggcggagactgcagtggagacaggctgccccctgatgatttgagtcatcacttgctgaggagcacctggctgtaccatcacaggtgttcgaataattgcctttcctagtgttgactgttggagtggtgttctaatcacggtcataccagggcgaatctgaggccctgtgattacttgtgaattgcttgtggttcctccagagcctgaggtattgggcctaattgtgactgttgctgtcctgggctggaatgaagtaaaggtttgctgactggtacctgtacttgatggaatgatacccaggactttctgctgtacttgaacaacgcctccttgtgttgctggcacatttacagcgacaatcttgctgtttgcaggaagtggcagtttggtaattacttttcctgccatagtgactggattgcctgtaatttggaacgtctgacctgtgctggcaatggttgtagcagatgtggcagctgtgctggtggctgaatttgactggccttgcttaacccatgtagcaaaggtttgatgaaagttcttgttttgttggaatgttactgtagctggagatccaactttagtagttagtaccattttggttccagttgtaactgagccacttatgggggccaccataaccttctgtgctggagagatggtgctggttgtactgcttgttggggaagtagtggaagttgcaatcactgtcggcttctgctgctccagtcgtttcttagcctgttgctcaactgcttgtgccttttctttctccactctctcagcaaatgccctgatctcccacaattccagttcttcttctgctacccaggtttcaataataacagggccagtttgcttgggcgtttctggtctctttggccgcagtgcacttgatcgaaggcctttcctctgaggtgtaggcgtttcttttggtgtttctggaactccaatgggacaaatgattttcctgatacaatattcagatcgaatgccataaggaccaacatctctcctcttaattatttctgttgttgtgatttcagtttcggatgtttctgtccgtgtagtccctcctcctggaggagccttggccgccatatcatcccatctcaaacttgcccacagtaaccgtaacatcaggctcactccagctaaggactttactgtctgaagtctatacctccaagtgatgccaaaggtcggtctaggagaaggatatggccatatatccaaagcaggttttgcattgtaattaaaataagggacctctcggattcctccttttcgggccaacttttttaagtcatcattaggcaaaacaaaaatgctcttcttgctgctcttggtaacaaattttctataggatggcagagctgtacctgaacgagtcttctttggtcttgaaaatttcatcagtttcactttgtctcgtgtggaatactctttgctcacagtcatagatgtaaccagtgtgcctcccgtggtggtcagggagtctgtcactgtcgtggtgaccacggttttgctctgctcctttacagagatgatgtccacactgccgcctgtggagggtgtggaaagcttggtcactgttgtagtggtggttgtgacagtggattttgcacaattttctgtggaagaaaccacagtttgcttatcgcctttttctaccttgatcacagtttttgattctgtggccactgtggaggtcatcgtggtgacttctgtgatgacggtttttcttttagattctccattgacattttcatttttgttgatgggcagaccattttcatcaataaagtcattactgagattagattcctcttcagaagtaataggtgatgaagtaactttcttaacttctgaggtttctatttccatatcttctacctgattaactgaattgctttctggacaagatgctgagggtgtggtcgtctgtgtactgtcagactctttggttgatggcagggtctcaaggctatctcggtagttaccttcagcatctgaagaactcagcaaatgcgattttgtttcggagctgtttctttcattaaaatcttccatgatgacatcaccattaatgaatggccttatagcagattctttaacagtcaatgatttaatatcattctcagggattattttatttatattattaacctttggttcaacattaccacttactactctactctcagaaatttctttcaagcattcacctttcaaatatattttgggtttattatcttttccatttatttgaaatgtacttgttctctgtcctttcttttcagactctcgattttcattattctttttgtcagtggtattttttagctttatttgatcactacatttattaactggtctctcctctaatttcttctgctgacttggttttttaccatttgcttcagtccccttgaccggcagcctgtcctcacagtttccagtggactcaccagaaaccaactcacactttaacggctccaagacttcaacatcttgttctcgagttctgaactgttcagaaatgctttcattgctattctgaacaatcatatcttcttcactgctatcctgaatagacacggtatcagaactattttccaaagtgctattagattcagagtcacatcccagttttccttcaaagtccattgctcttgacagaggtgtggcatctctgtcattggtacttttaggcactgatgaatgtaaagcactcttggaagaagaaacaatggtgtcactttcctcctgtatgagcggttttttgttcttacagatcaaagtaccaatatcatctgcactggctagtttagagtcatcgatgaaaaaatcatttccttttgttttactcttactgggttcctggcctctactggcaaggtcagagactttttcttctatgtcattttcaatggaattttgtttcggacattttgtttctgggctccgaatggagacatcatctaacactcgatcttttggataaagtttgtttgtggtatgactaggatcactcattctaagaactgaggaatcactttctgaacatccctgaatcaagtcctcaggttgatcattatttgcatttgggctctgttcttgtctcatcgagtcactctgacacccttcttttgctttcgttattactggtgattcagagagattttttgaagaatttgtagaagtctttcctatacccttaattccaccctccaacttgattttttcgagtcgctgtttttcttccagtgtaaactgtttaattctcctttcaagaagtccatctagtttggatgattttgttttctttttgtaactagtccttagatgaaaaccctcactaacattgaccacatctacttgagaactctcctgacaatttacatgtgactctgttttcatgtcatcgtctacttccattggttcttccttgcagggtttatcactgtcagaatctaagagctccttcacatcttggtccttcttctcagtaatctttgagatatccatttcattttggtctgctccttttgcagcatctgaaccttttacctcatctttttcagaatcaggctctatttttattttttttggacttcgtgaacattttcttttatctgactcatccatattttcatccatattatttttggttccttctaacgactttctgtaattcacattagtattgcctggcaatttaggaacaaacctataaacatgagttttactaatccagctccaaccaccatatcctgtcactctgtactcttcacctttttgtttccaaacctgatgcttaactggaaatgtgtattttacccatgtcgcttgctgcatcgtttcttcttcttcctgtttcttctctttttttttgactttctccttttcttctctttcaattgatgtcatccggtgtaacctggtatgtcctaaagattctcgccatattggtagcatcacaactggtttaactgcacactccaaaatggctaaagccaatgcaaattctctgggtttgctacacatctgaactgccttgatccaatttgccctatgtgatgcccagttgggatgaagaaaggatgaagggatgttgttttctaattgggtgatagtcagtctcagagtagatatggtaagaactttggacccatggacagaaccgttccatttgaactctcctgctggagtcagacagaacttatgtgcaagatgccttctcttatcatggtcttctctgtgctggtgcttattcaaagcaaatgaattggtggagtattgattgtggtagacgcgatacttcccttcttgacccaatttaaaataattgttgatatttcctttcatgatcacttcctttttggtgctcaaccgtgaaatttctccttgagagttaactaccagtacctctttgccctccttaaataatttatttgcttcatgtgcagcggctgccacctgctggctcttcagctgactaagtttgctatctggattccgcaatctggtgatgattcgagttgagccagatgctccttttccagctccaggagattcacttagctccccgttggacttctccgatttgaaatcaccctcagattttccttgctcagggtcatcatctggtgttttgtcgtcactgtctttttcaagggactggtcttcaaattcttctctgtttttctcagcatctttagagtcattctcagtctcattcttgtctttttctgtttcttctgggcttttaacattatcaatgtctccctttttggctcttatggattccaaaatttcttcattagctgccgccagaaaggatttgttactgccccgagccttattggtcaggtcttcagttatgtccatgtgtcggtggatttcttcacgcatttcttctagaattttgcagagttctgcttcccaataatctttgtctagacagtcaattaattctgcaagttggacctttgtgctgtaataccaaattttcttttcattttcattttctgtatcttcttctattatgagtcttcggttcaagaaccagtatttcctccgacttctatcatatccaataggttcatgtcgaatatatggtttatttttttggatttcagcaacacagtcagtcacaccaggcaccttgtgtgctacacagacttcacactgccactcgtcctctggcacctcctcaagaggtggcttcacacattccaaatggtatactgctgaacatgtctcacagcaaagcaaatccccaagtttgtgacaaaccctacaatggtcatcatactgtatcaccccttcagacatcaattcctctcgagcaatatttgttgtaagaaactgatcgactagaaactgtagaactttgatcttgttctctactggtccatatgggtagtcctctgcctcttggtaaggaagaacgtgatggtactccttatcactctcacagtacacccgcagcacctctggccacgtcatcccatctatgaaatacagtgtggaattaacgctatctttcagatcagcaggtccaaaggtagtattggaagtgtcttcttcacgcagaactgctttcaaaagcacaacatgcatctctgccatgagtgtgcactgctcttggctcaccagagctgcacaaaagtcctcaaagcgaaaaggagataatctcaaaacagtgccaaagttccgcagtacctcgtaaatggcaatgacattcattatatgctcattaggcaccattaaatcctcagaggacttgggaaattcaaggggcgggatgtctttttcttccaatataggagaacgaggccgatgtactcttggttttcgcctacctggagtgctgctgtaggtactatggctcctgaagctgctttccgtgcagtaactggcgtcgtcgtcgtcgtcttccatctcctccggataatcggagtcatcgtcgtcctcttccatctcatcctcctcgtcgtcctcagaatcctgggtctcctcggcgtcgccgtcctcctcctcctcctcctcggagaccatgtcctcctcttcctcctcctcctcgctctcgtggtcatcgtacaccactttgttgacggccctccgggccgcggtggtccgggccaggtggccgccgccgcccccgccccccgtcctgccgcccccgcctcctcgccccccccggcccggggcgctggtgctggggggggccggcggcggcggcggcggcttcctccggctactgctgccccccctgggcgagctcagccgcgtcttgggcgccacctcagcctgggcggcggcccacctgccccggctgctgccgcggtgccgcgagcggagccccccgatgggtccggacgtgggcggcggcggcggtggcggcggggccggggcgcagcgctccgcagcgggagccgcgggctgcttgggcggcctgccccgccggcccctcatgtcggagccgaggcggggggagaaggaaagcgaagggggaggggcgggcgcagggggggcggtggggagcgccggggccgggtggggaggcccgcggggccgggcgggaggggcccggccgacggaagcgggtggagggagaaggctcaatccgaattgctggggccccactccggatcgccttcagccgccatcttgtttcttccct

SEQ ID NO: 9362 - RNA, 8422 nt, Homo sapiens
  source 1..8422: mol_type = other RNA
aggaagccctggaggggctggaggagctggtgtcactggggggcagggtgcagctactgctgtggcctgagccaactgcatcaggtctttttctttcttaattttcaggtctctcttcagctcttcctgcacttcaatttgcagatccttgtccaggagtgctctcttcttcaggatctcggctctgagctgctctttgtgcttgaagagcagagctgacagcttagtggcattctgcttgctacgtttctgctccacactctcttcacgcttccgtttttttgctgcctgtttttcttctttatctatcttatccaaaatatacttcatcacctggttacagacaatcattctttgattctcttctctttcagctggagtcatgctctttttctgttttaaatgttctattacagcattatgcttcatcaccacctgtttctgaatgatttcactttgattagaagcttggagggtgtgttcacgcttaatttctatctgttgctgtttcttcttttgctgctgatccctgagttgctgaaccctttgcaactgctcttgcacactggctgcctgcactgtaaccacattctgaatctggtgagtctgcacagcactgctttgctgaatttggataggtaactggagtttgatttgctggggcacaccactttgctgagcctgtatctgagccacaacctgtgactggatctgagagagaacctggacttgttgttgcagctgaggcacagcaatgacttggggctgtggctgctgtatttgtagctgaggacgggatggggatgaaacagtaacttgatttaaagtttgtcctgatgaaagagtttgagttgaagactgtacctggggttgtgactgtggctggccttgggaaggtatctgaagagatgtatgtggttgaattggaatcggttgtgaggttgtagtctgaacctgggattgttgtccaggagacagttgggatggagttgatggacgtattcgagtctgtgatggactttggacacgaacaggagactgtccttggacattactttgaggctgagactgtgctgcaacttggggcttggatgactgtgcgtgggtgggttgtgcttcagaagggacatgggatgaaacagttgtttgggtctgaacttcaggctgagtctgaacttcaggctgagctggggactggggctgggtttggggctggggctgagctgaaggctgagcagtctgtggctgggcttctgctggacccacacttgatgactgagctggtggcagggttttgtcttgatgtacctgcatctggggtgacagtttactctgcctttgttcacctgtacctgctgctgtcgtggaaacagtggtggtggtggtgctggctgtggtggctgttgttgccaatggggtaaagaggaatcgctgaacagtaccatttggcattgcagcttgcattagctgctggcctgggcctgggagtacagtcaccccttgaggtatcaactgcaactgtccagtagtttgaccttgtccttgaattactactgtcaaaccttgattgccaccgtggccctgtgttaactgagtaagttgagccatggtgagcttcacttgtccttgttgggggcgagggggttgtgaggctgaagactgtatatttgaagtggacgttgctgaagttaagcttttctgcccaggtgttgaggaaaccgtgttaggggcggagactgcagtggagacaggctgccccctgatgatttgagtcatcacttgctgaggagcacctggctgtaccatcacaggtgttcgaataattgcctttcctagtgttgactgttggagtggtgttctaatcacggtcataccagggcgaatctgaggccctgtgattacttgtgaattgcttgtggttcctccagagcctgaggtattgggcctaattgtgactgttgctgtcctgggctggaatgaagtaaaggtttgctgactggtacctgtacttgatggaatgatacccaggactttctgctgtacttgaacaacgcctccttgtgttgctggcacatttacagcgacaatcttgctgtttgcaggaagtggcagtttggtaattacttttcctgccatagtgactggattgcctgtaatttggaacgtctgacctgtgctggcaatggttgtagcagatgtggcagctgtgctggtggctgaatttgactggccttgcttaacccatgtagcaaaggtttgatgaaagttcttgttttgttggaatgttactgtagctggagatccaactttagtagttagtaccattttggttccagttgtaactgagccacttatgggggccaccataaccttctgtgctggagagatggtgctggttgtactgcttgttggggaagtagtggaagttgcaatcactgtcggcttctgctgctccagtcgtttcttagcctgttgctcaactgcttgtgccttttctttctccactctctcagcaaatgccctgatctcccacaattccagttcttcttctgctacccaggtttcaataataacagggccagtttgcttgggcgtttctggtctctttggccgcagtgcacttgatcgaaggcctttcctctgaggtgtaggcgtttcttttggtgtttctggaactccaatgggacaaatgattttcctgatacaatattcagatcgaatgccataaggaccaacatctctcctcttaattatttctgttgttgtgatttcagtttcggatgtttctgtccgtgtagtccctcctcctggaggagccttggccgccatatcatcccatctcaaacttgcccacagtaaccgtaacatcaggctcactccagctaaggactttactgtctgaagtctatacctccaagtgatgccaaaggtcggtctaggagaaggatatggccatatatccaaagcaggttttgcattgtaattaaaataagggacctctcggattcctccttttcgggccaacttttttaagtcatcattaggcaaaacaaaaatgctcttcttgctgctcttggtaacaaattttctataggatggcagagctgtacctgaacgagtcttctttggtcttgaaaatttcatcagtttcactttgtctcgtgtggaatactctttgctcacagtcatagatgtaaccagtgtgcctcccgtggtggtcagggagtctgtcactgtcgtggtgaccacggttttgctctgctcctttacagagatgatgtccacactgccgcctgtggagggtgtggaaagcttggtcactgttgtagtggtggttgtgacagtggattttgcacaattttctgtggaagaaaccacagtttgcttatcgcctttttctaccttgatcacagtttttgattctgtggccactgtggaggtcatcgtggtgacttctgtgatgacggtttttcttttagattctccattgacattttcatttttgttgatgggcagaccattttcatcaataaagtcattactgagattagattcctcttcagaagtaataggtgatgaagtaactttcttaacttctgaggtttctatttccatatcttctacctgattaactgaattgctttctggacaagatgctgagggtgtggtcgtctgtgtactgtcagactctttggttgatggcagggtctcaaggctatctcggtagttaccttcagcatctgaagaactcagcaaatgcgattttgtttcggagctgtttctttcattaaaatcttccatgatgacatcaccattaatgaatggccttatagcagattctttaacagtcaatgatttaatatcattctcagggattattttatttatattattaacctttggttcaacattaccacttactactctactctcagaaatttctttcaagcattcacctttcaaatatattttgggtttattatcttttccatttatttgaaatgtacttgttctctgtcctttcttttcagactctcgattttcattattctttttgtcagtggtattttttagctttatttgatcactacatttattaactggtctctcctctaatttcttctgctgacttggttttttaccatttgcttcagtccccttgaccggcagcctgtcctcacagtttccagtggactcaccagaaaccaactcacactttaacggctccaagacttcaacatcttgttctcgagttctgaactgttcagaaatgctttcattgctattctgaacaatcatatcttcttcactgctatcctgaatagacacggtatcagaactattttccaaagtgctattagattcagagtcacatcccagttttccttcaaagtccattgctcttgacagaggtgtggcatctctgtcattggtacttttaggcactgatgaatgtaaagcactcttggaagaagaaacaatggtgtcactttcctcctgtatgagcggttttttgttcttacagatcaaagtaccaatatcatctgcactggctagtttagagtcatcgatgaaaaaatcatttccttttgttttactcttactgggttcctggcctctactggcaaggtcagagactttttcttctatgtcattttcaatggaattttgtttcggacattttgtttctgggctccgaatggagacatcatctaacactcgatcttttggataaagtttgtttgtggtatgactaggatcactcattctaagaactgaggaatcactttctgaacatccctgaatcaagtcctcaggttgatcattatttgcatttgggctctgttcttgtctcatcgagtcactctgacacccttcttttgctttcgttattactggtgattcagagagattttttgaagaatttgtagaagtctttcctatacccttaattccaccctccaacttgattttttcgagtcgctgtttttcttccagtgtaaactgtttaattctcctttcaagaagtccatctagtttggatgattttgttttctttttgtaactagtccttagatgaaaaccctcactaacattgaccacatctacttgagaactctcctgacaatttacatgtgactctgttttcatgtcatcgtctacttccattggttcttccttgcagggtttatcactgtcagaatctaagagctccttcacatcttggtccttcttctcagtaatctttgagatatccatttcattttggtctgctccttttgcagcatctgaaccttttacctcatctttttcagaatcaggctctatttttattttttttggacttcgtgaacattttcttttatctgactcatccatattttcatccatattatttttggttccttctaacgactttctgtaattcacattagtattgcctggcaatttaggaacaaacctataaacatgagttttactaatccagctccaaccaccatatcctgtcactctgtactcttcacctttttgtttccaaacctgatgcttaactggaaatgtgtattttacccatgtcgcttgctgcatcgtttcttcttcttcctgtttcttctctttttttttgactttctccttttcttctctttcaattgatgtcatccggtgtaacctggtatgtcctaaagattctcgccatattggtagcatcacaactggtttaactgcacactccaaaatggctaaagccaatgcaaattctctgggtttgctacacatctgaactgccttgatccaatttgccctatgtgatgcccagttgggatgaagaaaggatgaagggatgttgttttctaattgggtgatagtcagtctcagagtagatatggtaagaactttggacccatggacagaaccgttccatttgaactctcctgctggagtcagacagaacttatgtgcaagatgccttctcttatcatggtcttctctgtgctggtgcttattcaaagcaaatgaattggtggagtattgattgtggtagacgcgatacttcccttcttgacccaatttaaaataattgttgatatttcctttcatgatcacttcctttttggtgctcaaccgtgaaatttctccttgagagttaactaccagtacctctttgccctccttaaataatttatttgcttcatgtgcagcggctgccacctgctggctcttcagctgactaagtttgctatctggattccgcaatctggtgatgattcgagttgagccagatgctccttttccagctccaggagattcacttagctccccgttggacttctccgatttgaaatcacctacctcagattttccttgctcagggtcatcatctggtgttttgtcgtcactgtctttttcaagggactggtcttcaaattcttctctgtttttctcagcatctttagagtcattctcagtctcattcttgtctttttctgtttcttctgggcttttaacattatcaatgtctccctttttggctcttatggattccaaaatttcttcattagctgccgccagaaaggatttgttactgccccgagccttattggtcaggtcttcagttatgtccatgtgtcggtggatttcttcacgcatttcttctagaattttgcagagttctgcttcccaataatctttgtctagacagtcaattaattctgcaagttggacctttgtgctgtaataccaaattttcttttcattttcattttctgtatcttcttctattatgagtcttcggttcaagaaccagtatttcctccgacttctatcatatccaataggttcatgtcgaatatatggtttatttttttggatttcagcaacacagtcagtcacaccaggcaccttgtgtgctacacagacttcacactgccactcgtcctctggcacctcctcaagaggtggcttcacacattccaaatggtatactgctgaacatgtctcacagcaaagcaaatccccaagtttgtgacaaaccctacaatggtcatcatactgtatcaccccttcagacatcaattcctctcgagcaatatttgttgtaagaaactgatcgactagaaactgtagaactttgatcttgttctctactggtccatatgggtagtcctctgcctcttggtaaggaagaacgtgatggtactccttatcactctcacagtacacccgcagcacctctggccacgtcatcccatctatgaaatacagtgtggaattaacgctatctttcagatcagcaggtccaaaggtagtattggaagtgtcttcttcacgcagaactgctttcaaaagcacaacatgcatctctgccatgagtgtgcactgctcttggctcaccagagctgcacaaaagtcctcaaagcgaaaaggagataatctcaaaacagtgccaaagttccgcagtacctcgtaaatggcaatgacattcattatatgctcattaggcaccattaaatcctcagaggacttgggaaattcaaggggcgggatgtctttttcttccaatataggagaacgaggccgatgtactcttggttttcgcctacctggagtgctgctgtaggtactatggctcctgaagctgctttccgtgcagtaactggcgtcgtcgtcgtcgtcttccatctcctccggataatcggagtcatcgtcgtcctcttccatctcatcctcctcgtcgtcctcagaatcctgggtctcctcggcgtcgccgtcctcctcctcctcctcctcggagaccatgtcctcctcttcctcctcctcctcgctctcgtggtcatcgtacaccactttgttgacggccctccgggccgcggtggtccgggccaggtggccgccgccgcccccgccccccgtcctgccgcccccgcctcctcgccccccccggcccggggcgctggtgctggggggggccggcggcggcggcggcggcttcctccggctactgctgccccccctgggcgagctcagccgcgtcttgggcgccacctcagcctgggcggcggcccacctgccccggctgctgccgcggtgccgcgagcggagccccccgatgggtccggacgtgggcggcggcggcggtggcggcggggccggggcgcagcgctccgcagcgggagccgcgggctgcttgggcggcctgccccgccggcccctcatgtcggagccgaggcggggggagaaggaaagcgaagggggaggggcgggcgcagggggggcggtggggagcgccggggccgggtggggaggcccgcggggccgggcgggaggggcccggccgacggaagcgggtggagggagaaggctcaatccgaattgctggggccccactccggatcgccttcagccgccatcttgtttcttccct

SEQ ID NO: 9363 - RNA, 8608 nt, Homo sapiens
  source 1..8608: mol_type = other RNA
aggaagccctggaggggctggaggagctggtgtcactggggggcagggtgcagctactgctgtggcctgagccaactgcatcaggtctttttctttcttaattttcaggtctctcttcagctcttcctgcacttcaatttgcagatccttgtccaggagtgctctcttcttcaggatctcggctctgagctgctctttgtgcttgaagagcagagctgacagcttagtggcattctgcttgctacgtttctgctccacactctcttcacgcttccgtttttttgctgcctgtttttcttctttatctatcttatccaaaatatacttcatcacctggttacagacaatcattctttgattctcttctctttcagctggagtcatgctctttttctgttttaaatgttctattacagcattatgcttcatcaccacctgtttctgaatgatttcactttgattagaagcttggagggtgtgttcacgcttaatttctatctgttgctgtttcttcttttgctgctgatccctgagttgctgaaccctttgcaactgctcttgcacactggctgcctgcactgtaaccacattctgaatctggtgagtctgcacagcactgctttgctgaatttggataggtaactggagtttgatttgctggggcacaccactttgctgagcctgtatctgagccacaacctgtgactggatctgagagagaacctggacttgttgttgcagctgaggcacagcaatgacttggggctgtggctgctgtatttgtagctgaggacgggatggggatgaaacagtaacttgatttaaagtttgtcctgatgaaagagtttgagttgaagactgtacctggggttgtgactgtggctggccttgggaaggtatctgaagagatgtatgtggttgaattggaatcggttgtgaggttgtagtctgaacctgggattgttgtccaggagacagttgggatggagttgatggacgtattcgagtctgtgatggactttggacacgaacaggagactgtccttggacattactttgaggctgagactgtgctgcaacttggggcttggatgactgtgcgtgggtgggttgtgcttcagaagggacatgggatgaaacagttgtttgggtctgaacttcaggctgagtctgaacttcaggctgagctggggactggggctgggtttggggctggggctgagctgaaggctgagcagtctgtggctgggcttctgctggacccacacttgatgactgagctggtggcagggttttgtcttgatgtacctgcatctggggtgacagtttactctgcctttgttcacctgtacctgctgctgtcgtggaaacagtggtggtggtggtgctggctgtggtggctgttgttgccaatggggtaaagaggaatcgctgaacagtaccatttggcattgcagcttgcattagctgctggcctgggcctgggagtacagtcaccccttgaggtatcaactgcaactgtccagtagtttgaccttgtccttgaattactactgtcaaaccttgattgccaccgtggccctgtgttaactgagtaagttgagccatggtgagcttcacttgtccttgttgggggcgagggggttgtgaggctgaagactgtatatttgaagtggacgttgctgaagttaagcttttctgcccaggtgttgaggaaaccgtgttaggggcggagactgcagtggagacaggctgccccctgatgatttgagtcatcacttgctgaggagcacctggctgtaccatcacaggtgttcgaataattgcctttcctagtgttgactgttggagtggtgttctaatcacggtcataccagggcgaatctgaggccctgtgattacttgtgaattgcttgtggttcctccagagcctgaggtattgggcctaattgtgactgttgctgtcctgggctggaatgaagtaaaggtttgctgactggtacctgtacttgatggaatgatacccaggactttctgctgtacttgaacaacgcctccttgtgttgctggcacatttacagcgacaatcttgctgtttgcaggaagtggcagtttggtaattacttttcctgccatagtgactggattgcctgtaatttggaacgtctgacctgtgctggcaatggttgtagcagatgtggcagctgtgctggtggctgaatttgactggccttgcttaacccatgtagcaaaggtttgatgaaagttcttgttttgttggaatgttactgtagctggagatccaactttagtagttagtaccattttggttccagttgtaactgagccacttatgggggccaccataaccttctgtgctggagagatggtgctggttgtactgcttgttggggaagtagtggaagttgcaatcactgtcggcttctgctgctccagtcgtttcttagcctgttgctcaactgcttgtgccttttctttctccactctctcagcaaatgccctgatctcccacaattccagttcttcttctgctacccaggtttcaataataacagggccagtttgcttgggcgtttctggtctctttggccgcagtgcacttgatcgaaggcctttcctctgaggtgtaggcgtttcttttggtgtttctggaactccaatgggacaaatgattttcctgatacaatattcagatcgaatgccataaggaccaacatctctcctcttaattatttctgttgttgtgatttcagtttcggatgtttctgtccgtgtagtccctcctcctggaggagccttggccgccatatcatcccatctcaaacttgcccacagtaaccgtaacatcaggctcactccagctaaggactttactgtctgaagtctatacctccaagtgatgccaaaggtcggtctaggagaaggatatggccatatatccaaagcaggttttgcattgtaattaaaataagggacctctcggattcctccttttcgggccaacttttttaagtcatcattaggcaaaacaaaaatgctcttcttgctgctcttggtaacaaattttctataggatggcagagctgtacctgaacgagtcttctttggtcttgaaaatttcatcagtttcactttgtctcgtgtggaatactctttgctcacagtcatagatgtaaccagtgtgcctcccgtggtggtcagggagtctgtcactgtcgtggtgaccacggttttgctctgctcctttacagagatgatgtccacactgccgcctgtggagggtgtggaaagcttggtcactgttgtagtggtggttgtgacagtggattttgcacaattttctgtggaagaaaccacagtttgcttatcgcctttttctaccttgatcacagtttttgattctgtggccactgtggaggtcatcgtggtgacttctgtgatgacggtttttcttttagattctccattgacattttcatttttgttgatgggcagaccattttcatcaataaagtcattactgagattagattcctcttcagaagtaataggtgatgaagtaactttcttaacttctgaggtttctatttccatatcttctacctgattaactgaattgctttctggacaagatgctgagggtgtggtcgtctgtgtactgtcagactctttggttgatggcagggtctcaaggctatctcggtagttaccttcagcatctgaagaactcagcaaatgcgattttgtttcggagctgtttctttcattaaaatcttccatgatgacatcaccattaatgaatggccttatagcagattctttaacagtcaatgatttaatatcattctcagggattattttatttatattattaacctttggttcaacattaccacttactactctactctcagaaatttctttcaagcattcacctttcaaatatattttgggtttattatcttttccatttatttgaaatgtacttgttctctgtcctttcttttcagactctcgattttcattattctttttgtcagtggtattttttagctttatttgatcactacatttattaactggtctctcctctaatttcttctgctgacttggttttttaccatttgcttcagtccccttgaccggcagcctgtcctcacagtttccagtggactcaccagaaaccaactcacactttaacggctccaagacttcaacatcttgttctcgagttctgaactgttcagaaatgctttcattgctattctgaacaatcatatcttcttcactgctatcctgaatagacacggtatcagaactattttccaaagtgctattagattcagagtcacatcccagttttccttcaaagtccattgctcttgacagaggtgtggcatctctgtcattggtacttttaggcactgatgaatgtaaagcactcttggaagaagaaacaatggtgtcactttcctcctgtatgagcggttttttgttcttacagatcaaagtaccaatatcatctgcactggctagtttagagtcatcgatgaaaaaatcatttccttttgttttactcttactgggttcctggcctctactggcaaggtcagagactttttcttctatgtcattttcaatggaattttgtttcggacattttgtttctgggctccgaatggagacatcatctaacactcgatcttttggataaagtttgtttgtggtatgactaggatcactcattctaagaactgaggaatcactttctgaacatccctgaatcaagtcctcaggttgatcattatttgcatttgggctctgttcttgtctcatcgagtcactctgacacccttcttttgctttcgttattactggtgattcagagagattttttgaagaatttgtagaagtctttcctatacccttaattccaccctccaacttgattttttcgagtcgctgtttttcttccagtgtaaactgtttaattctcctttcaagaagtccatctagtttggatgattttgttttctttttgtaactagtccttagatgaaaaccctcactaacattgaccacatctacttgagaactctcctgacaatttacatgtgactctgttttcatgtcatcgtctacttccattggttcttccttgcagggtttatcactgtcagaatctaagagctccttcacatcttggtccttcttctcagtaatctttgagatatccatttcattttggtctgctccttttgcagcatctgaaccttttacctcatctttttcagaatcaggctctatttttattttttttggacttcgtgaacattttcttttatctgactcatccatattttcatccatattatttttggttccttctaacgactttctgtaattcacattagtattgcctggcaatttaggaacaaacctataaacatgagttttactaatccagctccaaccaccatatcctgtcactctgtactcttcacctttttgtttccaaacctgatgcttaactggaaatgtgtattttacccatgtcgcttgctgcatcgtttcttcttcttcctgtttcttctctttttttttgactttctccttttcttctctttcaattgatgtcatccggtgtaacctggtatgtcctaaagattctcgccatattggtagcatcacaactggtttaactgcacactccaaaatggctaaagccaatgcaaattctctgggtttgctacacatctgaactgccttgatccaatttgccctatgtgatgcccagttgggatgaagaaaggatgaagggatgttgttttctaattgggtgatagtcagtctcagagtagatatggtaagaactttggacccatggacagaaccgttccatttgaactctcctgctggagtcagacagaacttatgtgcaagatgccttctcttatcatggtcttctctgtgctggtgcttattcaaagcaaatgaattggtggagtattgattgtggtagacgcgatacttcccttcttgacccaatttaaaataattgttgatatttcctttcatgatcacttcctttttggtgctcaaccgtgaaatttctccttgagagttaactaccagtacctctttgccctccttaaataatttatttgcttcatgtgcagcggctgccacctgctggctcttcagctgactaagtttgctatctggattccgcaatctggtgatgattcgagttgagccagatgctccttttccagctccaggagattcacttagctccccgttggacttctccgatttgaaatcacctactatctcttcctgaatagagacaggtgtatgagattctctttctccattttcaggatcatcagctgccttagcagattcactctgggaagaatttagttcactgctgctgttactgttttccagattaggctggatggaggtagtggtagcactagtgttactgctctcacatgtcttgttaggttcctcagattttccttgctcagggtcatcatctggtgttttgtcgtcactgtctttttcaagggactggtcttcaaattcttctctgtttttctcagcatctttagagtcattctcagtctcattcttgtctttttctgtttcttctgggcttttaacattatcaatgtctccctttttggctcttatggattccaaaatttcttcattagctgccgccagaaaggatttgttactgccccgagccttattggtcaggtcttcagttatgtccatgtgtcggtggatttcttcacgcatttcttctagaattttgcagagttctgcttcccaataatctttgtctagacagtcaattaattctgcaagttggacctttgtgctgtaataccaaattttcttttcattttcattttctgtatcttcttctattatgagtcttcggttcaagaaccagtatttcctccgacttctatcatatccaataggttcatgtcgaatatatggtttatttttttggatttcagcaacacagtcagtcacaccaggcaccttgtgtgctacacagacttcacactgccactcgtcctctggcacctcctcaagaggtggcttcacacattccaaatggtatactgctgaacatgtctcacagcaaagcaaatccccaagtttgtgacaaaccctacaatggtcatcatactgtatcaccccttcagacatcaattcctctcgagcaatatttgttgtaagaaactgatcgactagaaactgtagaactttgatcttgttctctactggtccatatgggtagtcctctgcctcttggtaaggaagaacgtgatggtactccttatcactctcacagtacacccgcagcacctctggccacgtcatcccatctatgaaatacagtgtggaattaacgctatctttcagatcagcaggtccaaaggtagtattggaagtgtcttcttcacgcagaactgctttcaaaagcacaacatgcatctctgccatgagtgtgcactgctcttggctcaccagagctgcacaaaagtcctcaaagcgaaaaggagataatctcaaaacagtgccaaagttccgcagtacctcgtaaatggcaatgacattcattatatgctcattaggcaccattaaatcctcagaggacttgggaaattcaaggggcgggatgtctttttcttccaatataggagaacgaggccgatgtactcttggttttcgcctacctggagtgctgctgtaggtactatggctcctgaagctgctttccgtgcagtaactggcgtcgtcgtcgtcgtcttccatctcctccggataatcggagtcatcgtcgtcctcttccatctcatcctcctcgtcgtcctcagaatcctgggtctcctcggcgtcgccgtcctcctcctcctcctcctcggagaccatgtcctcctcttcctcctcctcctcgctctcgtggtcatcgtacaccactttgttgacggccctccgggccgcggtggtccgggccaggtggccgccgccgcccccgccccccgtcctgccgcccccgcctcctcgccccccccggcccggggcgctggtgctggggggggccggcggcggcggcggcggcttcctccggctactgctgccccccctgggcgagctcagccgcgtcttgggcgccacctcagcctgggcggcggcccacctgccccggctgctgccgcggtgccgcgagcggagccccccgatgggtccggacgtgggcggcggcggcggtggcggcggggccggggcgcagcgctccgcagcgggagccgcgggctgcttgggcggcctgccccgccggcccctcatgtcggagccgaggcggggggagaaggaaagcgaagggggaggggcgggcgcagggggggcggtggggagcgccggggccgggtggggaggcccgcggggccgggcgggaggggcccggccgacggaagcgggtggagggagaaggctcaatccgaattgctggggccccactccggatcgccttcagccgccatcttgtttcttccct

SEQ ID NO: 9364 - RNA, 8797 nt, Homo sapiens
  source 1..8797: mol_type = other RNA
aggaagccctggaggggctggaggagctggtgtcactggggggcagggtgcagctactgctgtggcctgagccaactgcatcaggtctttttctttcttaattttcaggtctctcttcagctcttcctgcacttcaatttgcagatccttgtccaggagtgctctcttcttcaggatctcggctctgagctgctctttgtgcttgaagagcagagctgacagcttagtggcattctgcttgctacgtttctgctccacactctcttcacgcttccgtttttttgctgcctgtttttcttctttatctatcttatccaaaatatacttcatcacctggttacagacaatcattctttgattctcttctctttcagctggagtcatgctctttttctgttttaaatgttctattacagcattatgcttcatcaccacctgtttctgaatgatttcactttgattagaagcttggagggtgtgttcacgcttaatttctatctgttgctgtttcttcttttgctgctgatccctgagttgctgaaccctttgcaactgctcttgcacactggctgcctgcactgtaaccacattctgaatctggtgagtctgcacagcactgctttgctgaatttggataggtaactggagtttgatttgctggggcacaccactttgctgagcctgtatctgagccacaacctgtgactggatctgagagagaacctggacttgttgttgcagctgaggcacagcaatgacttggggctgtggctgctgtatttgtagctgaggacgggatggggatgaaacagtaacttgatttaaagtttgtcctgatgaaagagtttgagttgaagactgtacctggggttgtgactgtggctggccttgggaaggtatctgaagagatgtatgtggttgaattggaatcggttgtgaggttgtagtctgaacctgggattgttgtccaggagacagttgggatggagttgatggacgtattcgagtctgtgatggactttggacacgaacaggagactgtccttggacattactttgaggctgagactgtgctgcaacttggggcttggatgactgtgcgtgggtgggttgtgcttcagaagggacatgggatgaaacagttgtttgggtctgaacttcaggctgagtctgaacttcaggctgagctggggactggggctgggtttggggctggggctgagctgaaggctgagcagtctgtggctgggcttctgctggacccacacttgatgactgagctggtggcagggttttgtcttgatgtacctgcatctggggtgacagtttactctgcctttgttcacctgtacctgctgctgtcgtggaaacagtggtggtggtggtgctggctgtggtggctgttgttgccaatggggtaaagaggaatcgctgaacagtaccatttggcattgcagcttgcattagctgctggcctgggcctgggagtacagtcaccccttgaggtatcaactgcaactgtccagtagtttgaccttgtccttgaattactactgtcaaaccttgattgccaccgtggccctgtgttaactgagtaagttgagccatggtgagcttcacttgtccttgttgggggcgagggggttgtgaggctgaagactgtatatttgaagtggacgttgctgaagttaagcttttctgcccaggtgttgaggaaaccgtgttaggggcggagactgcagtggagacaggctgccccctgatgatttgagtcatcacttgctgaggagcacctggctgtaccatcacaggtgttcgaataattgcctttcctagtgttgactgttggagtggtgttctaatcacggtcataccagggcgaatctgaggccctgtgattacttgtgaattgcttgtggttcctccagagcctgaggtattgggcctaattgtgactgttgctgtcctgggctggaatgaagtaaaggtttgctgactggtacctgtacttgatggaatgatacccaggactttctgctgtacttgaacaacgcctccttgtgttgctggcacatttacagcgacaatcttgctgtttgcaggaagtggcagtttggtaattacttttcctgccatagtgactggattgcctgtaatttggaacgtctgacctgtgctggcaatggttgtagcagatgtggcagctgtgctggtggctgaatttgactggccttgcttaacccatgtagcaaaggtttgatgaaagttcttgttttgttggaatgttactgtagctggagatccaactttagtagttagtaccattttggttccagttgtaactgagccacttatgggggccaccataaccttctgtgctggagagatggtgctggttgtactgcttgttggggaagtagtggaagttgcaatcactgtcggcttctgctgctccagtcgtttcttagcctgttgctcaactgcttgtgccttttctttctccactctctcagcaaatgccctgatctcccacaattccagttcttcttctgctacccaggtttcaataataacagggccagtttgcttgggcgtttctggtctctttggccgcagtgcacttgatcgaaggcctttcctctgaggtgtaggcgtttcttttggtgtttctggaactccaatgggacaaatgattttcctgatacaatattcagatcgaatgccataaggaccaacatctctcctcttaattatttctgttgttgtgatttcagtttcggatgtttctgtccgtgtagtccctcctcctggaggagccttggccgccatatcatcccatctcaaacttgcccacagtaaccgtaacatcaggctcactccagctaaggactttactgtctgaagtctatacctccaagtgatgccaaaggtcggtctaggagaaggatatggccatatatccaaagcaggttttgcattgtaattaaaataagggacctctcggattcctccttttcgggccaacttttttaagtcatcattaggcaaaacaaaaatgctcttcttgctgctcttggtaacaaattttctataggatggcagagctgtacctgaacgagtcttctttggtcttgaaaatttcatcagtttcactttgtctcgtgtggaatactctttgctcacagtcatagatgtaaccagtgtgcctcccgtggtggtcagggagtctgtcactgtcgtggtgaccacggttttgctctgctcctttacagagatgatgtccacactgccgcctgtggagggtgtggaaagcttggtcactgttgtagtggtggttgtgacagtggattttgcacaattttctgtggaagaaaccacagtttgcttatcgcctttttctaccttgatcacagtttttgattctgtggccactgtggaggtcatcgtggtgacttctgtgatgacggtttttcttttagattctccattgacattttcatttttgttgatgggcagaccattttcatcaataaagtcattactgagattagattcctcttcagaagtaataggtgatgaagtaactttcttaacttctgaggtttctatttccatatcttctacctgattaactgaattgctttctggacaagatgctgagggtgtggtcgtctgtgtactgtcagactctttggttgatggcagggtctcaaggctatctcggtagttaccttcagcatctgaagaactcagcaaatgcgattttgtttcggagctgtttctttcattaaaatcttccatgatgacatcaccattaatgaatggccttatagcagattctttaacagtcaatgatttaatatcattctcagggattattttatttatattattaacctttggttcaacattaccacttactactctactctcagaaatttctttcaagcattcacctttcaaatatattttgggtttattatcttttccatttatttgaaatgtacttgttctctgtcctttcttttcagactctcgattttcattattctttttgtcagtggtattttttagctttatttgatcactacatttattaactggtctctcctctaatttcttctgctgacttggttttttaccatttgcttcagtccccttgaccggcagcctgtcctcacagtttccagtggactcaccagaaaccaactcacactttaacggctccaagacttcaacatcttgttctcgagttctgaactgttcagaaatgctttcattgctattctgaacaatcatatcttcttcactgctatcctgaatagacacggtatcagaactattttccaaagtgctattagattcagagtcacatcccagttttccttcaaagtccattgctcttgacagaggtgtggcatctctgtcattggtacttttaggcactgatgaatgtaaagcactcttggaagaagaaacaatggtgtcactttcctcctgtatgagcggttttttgttcttacagatcaaagtaccaatatcatctgcactggctagtttagagtcatcgatgaaaaaatcatttccttttgttttactcttactgggttcctggcctctactggcaaggtcagagactttttcttctatgtcattttcaatggaattttgtttcggacattttgtttctgggctccgaatggagacatcatctaacactcgatcttttggataaagtttgtttgtggtatgactaggatcactcattctaagaactgaggaatcactttctgaacatccctgaatcaagtcctcaggttgatcattatttgcatttgggctctgttcttgtctcatcgagtcactctgacacccttcttttgctttcgttattactggtgattcagagagattttttgaagaatttgtagaagtctttcctatacccttaattccaccctccaacttgattttttcgagtcgctgtttttcttccagtgtaaactgtttaattctcctttcaagaagtccatctagtttggatgattttgttttctttttgtaactagtccttagatgaaaaccctcactaacattgaccacatctacttgagaactctcctgacaatttacatgtgactctgttttcatgtcatcgtctacttccattggttcttccttgcagggtttatcactgtcagaatctaagagctccttcacatcttggtccttcttctcagtaatctttgagatatccatttcattttggtctgctccttttgcagcatctgaaccttttacctcatctttttcagaatcaggctctatttttattttttttggacttcgtgaacattttcttttatctgactcatccatattttcatccatattatttttggttccttctaacgactttctgtaattcacattagtattgcctggcaatttaggaacaaacctataaacatgagttttactaatccagctccaaccaccatatcctgtcactctgtactcttcacctttttgtttccaaacctgatgcttaactggaaatgtgtattttacccatgtcgcttgctgcatcgtttcttcttcttcctgtttcttctctttttttttgactttctccttttcttctctttcaattgatgtcatccggtgtaacctggtatgtcctaaagattctcgccatattggtagcatcacaactggtttaactgcacactccaaaatggctaaagccaatgcaaattctctgggtttgctacacatctgaactgccttgatccaatttgccctatgtgatgcccagttgggatgaagaaaggatgaagggatgttgttttctaattgggtgatagtcagtctcagagtagatatggtaagaactttggacccatggacagaaccgttccatttgaactctcctgctggagtcagacagaacttatgtgcaagatgccttctcttatcatggtcttctctgtgctggtgcttattcaaagcaaatgaattggtggagtattgattgtggtagacgcgatacttcccttcttgacccaatttaaaataattgttgatatttcctttcatgatcacttcctttttggtgctcaaccgtgaaatttctccttgagagttaactaccagtacctctttgccctccttaaataatttatttgcttcatgtgcagcggctgccacctgctggctcttcagctgactaagtttgctatctggattccgcaatctggtgatgattcgagttgagccagatgctccttttccagctccaggagattcacttagctccccgttggacttctccgatttgaaatcacctactatctcttcctgaatagagacaggtgtatgagattctctttctccattttcaggatcatcagctgccttagcagattcactctgggaagaatttagttcactgctgctgttactgttttccagattaggctggatggaggtagtggtagcactagtgttactgctctcacatgtcttgttaggttctggcacatcctgggggagctcagatgccaccttcttctctgccatgttgctgctatcgggggtttctgagagacaccccacagggctcctcccttcagagggactagtctcttctgaagttgcatttgttgtgttgtcgccaagatttgctgacacagagttacctttatccccaacttctgttggctcctcagattttccttgctcagggtcatcatctggtgttttgtcgtcactgtctttttcaagggactggtcttcaaattcttctctgtttttctcagcatctttagagtcattctcagtctcattcttgtctttttctgtttcttctgggcttttaacattatcaatgtctccctttttggctcttatggattccaaaatttcttcattagctgccgccagaaaggatttgttactgccccgagccttattggtcaggtcttcagttatgtccatgtgtcggtggatttcttcacgcatttcttctagaattttgcagagttctgcttcccaataatctttgtctagacagtcaattaattctgcaagttggacctttgtgctgtaataccaaattttcttttcattttcattttctgtatcttcttctattatgagtcttcggttcaagaaccagtatttcctccgacttctatcatatccaataggttcatgtcgaatatatggtttatttttttggatttcagcaacacagtcagtcacaccaggcaccttgtgtgctacacagacttcacactgccactcgtcctctggcacctcctcaagaggtggcttcacacattccaaatggtatactgctgaacatgtctcacagcaaagcaaatccccaagtttgtgacaaaccctacaatggtcatcatactgtatcaccccttcagacatcaattcctctcgagcaatatttgttgtaagaaactgatcgactagaaactgtagaactttgatcttgttctctactggtccatatgggtagtcctctgcctcttggtaaggaagaacgtgatggtactccttatcactctcacagtacacccgcagcacctctggccacgtcatcccatctatgaaatacagtgtggaattaacgctatctttcagatcagcaggtccaaaggtagtattggaagtgtcttcttcacgcagaactgctttcaaaagcacaacatgcatctctgccatgagtgtgcactgctcttggctcaccagagctgcacaaaagtcctcaaagcgaaaaggagataatctcaaaacagtgccaaagttccgcagtacctcgtaaatggcaatgacattcattatatgctcattaggcaccattaaatcctcagaggacttgggaaattcaaggggcgggatgtctttttcttccaatataggagaacgaggccgatgtactcttggttttcgcctacctggagtgctgctgtaggtactatggctcctgaagctgctttccgtgcagtaactggcgtcgtcgtcgtcgtcttccatctcctccggataatcggagtcatcgtcgtcctcttccatctcatcctcctcgtcgtcctcagaatcctgggtctcctcggcgtcgccgtcctcctcctcctcctcctcggagaccatgtcctcctcttcctcctcctcctcgctctcgtggtcatcgtacaccactttgttgacggccctccgggccgcggtggtccgggccaggtggccgccgccgcccccgccccccgtcctgccgcccccgcctcctcgccccccccggcccggggcgctggtgctggggggggccggcggcggcggcggcggcttcctccggctactgctgccccccctgggcgagctcagccgcgtcttgggcgccacctcagcctgggcggcggcccacctgccccggctgctgccgcggtgccgcgagcggagccccccgatgggtccggacgtgggcggcggcggcggtggcggcggggccggggcgcagcgctccgcagcgggagccgcgggctgcttgggcggcctgccccgccggcccctcatgtcggagccgaggcggggggagaaggaaagcgaagggggaggggcgggcgcagggggggcggtggggagcgccggggccgggtggggaggcccgcggggccgggcgggaggggcccggccgacggaagcgggtggagggagaaggctcaatccgaattgctggggccccactccggatcgccttcagccgccatcttgtttcttccct

SEQ ID NO: 9365 - RNA, 8611 nt, Homo sapiens
  source 1..8611: mol_type = other RNA
aggaagccctggaggggctggaggagctggtgtcactggggggcagggtgcagctactgctgtggcctgagccaactgcatcaggtctttttctttcttaattttcaggtctctcttcagctcttcctgcacttcaatttgcagatccttgtccaggagtgctctcttcttcaggatctcggctctgagctgctctttgtgcttgaagagcagagctgacagcttagtggcattctgcttgctacgtttctgctccacactctcttcacgcttccgtttttttgctgcctgtttttcttctttatctatcttatccaaaatatacttcatcacctggttacagacaatcattctttgattctcttctctttcagctggagtcatgctctttttctgttttaaatgttctattacagcattatgcttcatcaccacctgtttctgaatgatttcactttgattagaagcttggagggtgtgttcacgcttaatttctatctgttgctgtttcttcttttgctgctgatccctgagttgctgaaccctttgcaactgctcttgcacactggctgcctgcactgtaaccacattctgaatctggtgagtctgcacagcactgctttgctgaatttggataggtaactggagtttgatttgctggggcacaccactttgctgagcctgtatctgagccacaacctgtgactggatctgagagagaacctggacttgttgttgcagctgaggcacagcaatgacttggggctgtggctgctgtatttgtagctgaggacgggatggggatgaaacagtaacttgatttaaagtttgtcctgatgaaagagtttgagttgaagactgtacctggggttgtgactgtggctggccttgggaaggtatctgaagagatgtatgtggttgaattggaatcggttgtgaggttgtagtctgaacctgggattgttgtccaggagacagttgggatggagttgatggacgtattcgagtctgtgatggactttggacacgaacaggagactgtccttggacattactttgaggctgagactgtgctgcaacttggggcttggatgactgtgcgtgggtgggttgtgcttcagaagggacatgggatgaaacagttgtttgggtctgaacttcaggctgagtctgaacttcaggctgagctggggactggggctgggtttggggctggggctgagctgaaggctgagcagtctgtggctgggcttctgctggacccacacttgatgactgagctggtggcagggttttgtcttgatgtacctgcatctggggtgacagtttactctgcctttgttcacctgtacctgctgctgtcgtggaaacagtggtggtggtggtgctggctgtggtggctgttgttgccaatggggtaaagaggaatcgctgaacagtaccatttggcattgcagcttgcattagctgctggcctgggcctgggagtacagtcaccccttgaggtatcaactgcaactgtccagtagtttgaccttgtccttgaattactactgtcaaaccttgattgccaccgtggccctgtgttaactgagtaagttgagccatggtgagcttcacttgtccttgttgggggcgagggggttgtgaggctgaagactgtatatttgaagtggacgttgctgaagttaagcttttctgcccaggtgttgaggaaaccgtgttaggggcggagactgcagtggagacaggctgccccctgatgatttgagtcatcacttgctgaggagcacctggctgtaccatcacaggtgttcgaataattgcctttcctagtgttgactgttggagtggtgttctaatcacggtcataccagggcgaatctgaggccctgtgattacttgtgaattgcttgtggttcctccagagcctgaggtattgggcctaattgtgactgttgctgtcctgggctggaatgaagtaaaggtttgctgactggtacctgtacttgatggaatgatacccaggactttctgctgtacttgaacaacgcctccttgtgttgctggcacatttacagcgacaatcttgctgtttgcaggaagtggcagtttggtaattacttttcctgccatagtgactggattgcctgtaatttggaacgtctgacctgtgctggcaatggttgtagcagatgtggcagctgtgctggtggctgaatttgactggccttgcttaacccatgtagcaaaggtttgatgaaagttcttgttttgttggaatgttactgtagctggagatccaactttagtagttagtaccattttggttccagttgtaactgagccacttatgggggccaccataaccttctgtgctggagagatggtgctggttgtactgcttgttggggaagtagtggaagttgcaatcactgtcggcttctgctgctccagtcgtttcttagcctgttgctcaactgcttgtgccttttctttctccactctctcagcaaatgccctgatctcccacaattccagttcttcttctgctacccaggtttcaataataacagggccagtttgcttgggcgtttctggtctctttggccgcagtgcacttgatcgaaggcctttcctctgaggtgtaggcgtttcttttggtgtttctggaactccaatgggacaaatgattttcctgatacaatattcagatcgaatgccataaggaccaacatctctcctcttaattatttctgttgttgtgatttcagtttcggatgtttctgtccgtgtagtccctcctcctggaggagccttggccgccatatcatcccatctcaaacttgcccacagtaaccgtaacatcaggctcactccagctaaggactttactgtctgaagtctatacctccaagtgatgccaaaggtcggtctaggagaaggatatggccatatatccaaagcaggttttgcattgtaattaaaataagggacctctcggattcctccttttcgggccaacttttttaagtcatcattaggcaaaacaaaaatgctcttcttgctgctcttggtaacaaattttctataggatggcagagctgtacctgaacgagtcttctttggtcttgaaaatttcatcagtttcactttgtctcgtgtggaatactctttgctcacagtcatagatgtaaccagtgtgcctcccgtggtggtcagggagtctgtcactgtcgtggtgaccacggttttgctctgctcctttacagagatgatgtccacactgccgcctgtggagggtgtggaaagcttggtcactgttgtagtggtggttgtgacagtggattttgcacaattttctgtggaagaaaccacagtttgcttatcgcctttttctaccttgatcacagtttttgattctgtggccactgtggaggtcatcgtggtgacttctgtgatgacggtttttcttttagattctccattgacattttcatttttgttgatgggcagaccattttcatcaataaagtcattactgagattagattcctcttcagaagtaataggtgatgaagtaactttcttaacttctgaggtttctatttccatatcttctacctgattaactgaattgctttctggacaagatgctgagggtgtggtcgtctgtgtactgtcagactctttggttgatggcagggtctcaaggctatctcggtagttaccttcagcatctgaagaactcagcaaatgcgattttgtttcggagctgtttctttcattaaaatcttccatgatgacatcaccattaatgaatggccttatagcagattctttaacagtcaatgatttaatatcattctcagggattattttatttatattattaacctttggttcaacattaccacttactactctactctcagaaatttctttcaagcattcacctttcaaatatattttgggtttattatcttttccatttatttgaaatgtacttgttctctgtcctttcttttcagactctcgattttcattattctttttgtcagtggtattttttagctttatttgatcactacatttattaactggtctctcctctaatttcttctgctgacttggttttttaccatttgcttcagtccccttgaccggcagcctgtcctcacagtttccagtggactcaccagaaaccaactcacactttaacggctccaagacttcaacatcttgttctcgagttctgaactgttcagaaatgctttcattgctattctgaacaatcatatcttcttcactgctatcctgaatagacacggtatcagaactattttccaaagtgctattagattcagagtcacatcccagttttccttcaaagtccattgctcttgacagaggtgtggcatctctgtcattggtacttttaggcactgatgaatgtaaagcactcttggaagaagaaacaatggtgtcactttcctcctgtatgagcggttttttgttcttacagatcaaagtaccaatatcatctgcactggctagtttagagtcatcgatgaaaaaatcatttccttttgttttactcttactgggttcctggcctctactggcaaggtcagagactttttcttctatgtcattttcaatggaattttgtttcggacattttgtttctgggctccgaatggagacatcatctaacactcgatcttttggataaagtttgtttgtggtatgactaggatcactcattctaagaactgaggaatcactttctgaacatccctgaatcaagtcctcaggttgatcattatttgcatttgggctctgttcttgtctcatcgagtcactctgacacccttcttttgctttcgttattactggtgattcagagagattttttgaagaatttgtagaagtctttcctatacccttaattccaccctccaacttgattttttcgagtcgctgtttttcttccagtgtaaactgtttaattctcctttcaagaagtccatctagtttggatgattttgttttctttttgtaactagtccttagatgaaaaccctcactaacattgaccacatctacttgagaactctcctgacaatttacatgtgactctgttttcatgtcatcgtctacttccattggttcttccttgcagggtttatcactgtcagaatctaagagctccttcacatcttggtccttcttctcagtaatctttgagatatccatttcattttggtctgctccttttgcagcatctgaaccttttacctcatctttttcagaatcaggctctatttttattttttttggacttcgtgaacattttcttttatctgactcatccatattttcatccatattatttttggttccttctaacgactttctgtaattcacattagtattgcctggcaatttaggaacaaacctataaacatgagttttactaatccagctccaaccaccatatcctgtcactctgtactcttcacctttttgtttccaaacctgatgcttaactggaaatgtgtattttacccatgtcgcttgctgcatcgtttcttcttcttcctgtttcttctctttttttttgactttctccttttcttctctttcaattgatgtcatccggtgtaacctggtatgtcctaaagattctcgccatattggtagcatcacaactggtttaactgcacactccaaaatggctaaagccaatgcaaattctctgggtttgctacacatctgaactgccttgatccaatttgccctatgtgatgcccagttgggatgaagaaaggatgaagggatgttgttttctaattgggtgatagtcagtctcagagtagatatggtaagaactttggacccatggacagaaccgttccatttgaactctcctgctggagtcagacagaacttatgtgcaagatgccttctcttatcatggtcttctctgtgctggtgcttattcaaagcaaatgaattggtggagtattgattgtggtagacgcgatacttcccttcttgacccaatttaaaataattgttgatatttcctttcatgatcacttcctttttggtgctcaaccgtgaaatttctccttgagagttaactaccagtacctctttgccctccttaaataatttatttgcttcatgtgcagcggctgccacctgctggctcttcagctgactaagtttgctatctggattccgcaatctggtgatgattcgagttgagccagatgctccttttccagctccaggagattcacttagctccccgttggacttctccgatttgaaatcacctactatctcttcctgaatagagacaggtgtatgagattctctttctccattttcaggatcatcagctgccttagcagattcactctgggaagaatttagttcactgctgctgttactgttttccagattaggctggatggaggtagtggtagcactagtgttactgctctcacatgtcttgttaggttcttcctcagattttccttgctcagggtcatcatctggtgttttgtcgtcactgtctttttcaagggactggtcttcaaattcttctctgtttttctcagcatctttagagtcattctcagtctcattcttgtctttttctgtttcttctgggcttttaacattatcaatgtctccctttttggctcttatggattccaaaatttcttcattagctgccgccagaaaggatttgttactgccccgagccttattggtcaggtcttcagttatgtccatgtgtcggtggatttcttcacgcatttcttctagaattttgcagagttctgcttcccaataatctttgtctagacagtcaattaattctgcaagttggacctttgtgctgtaataccaaattttcttttcattttcattttctgtatcttcttctattatgagtcttcggttcaagaaccagtatttcctccgacttctatcatatccaataggttcatgtcgaatatatggtttatttttttggatttcagcaacacagtcagtcacaccaggcaccttgtgtgctacacagacttcacactgccactcgtcctctggcacctcctcaagaggtggcttcacacattccaaatggtatactgctgaacatgtctcacagcaaagcaaatccccaagtttgtgacaaaccctacaatggtcatcatactgtatcaccccttcagacatcaattcctctcgagcaatatttgttgtaagaaactgatcgactagaaactgtagaactttgatcttgttctctactggtccatatgggtagtcctctgcctcttggtaaggaagaacgtgatggtactccttatcactctcacagtacacccgcagcacctctggccacgtcatcccatctatgaaatacagtgtggaattaacgctatctttcagatcagcaggtccaaaggtagtattggaagtgtcttcttcacgcagaactgctttcaaaagcacaacatgcatctctgccatgagtgtgcactgctcttggctcaccagagctgcacaaaagtcctcaaagcgaaaaggagataatctcaaaacagtgccaaagttccgcagtacctcgtaaatggcaatgacattcattatatgctcattaggcaccattaaatcctcagaggacttgggaaattcaaggggcgggatgtctttttcttccaatataggagaacgaggccgatgtactcttggttttcgcctacctggagtgctgctgtaggtactatggctcctgaagctgctttccgtgcagtaactggcgtcgtcgtcgtcgtcttccatctcctccggataatcggagtcatcgtcgtcctcttccatctcatcctcctcgtcgtcctcagaatcctgggtctcctcggcgtcgccgtcctcctcctcctcctcctcggagaccatgtcctcctcttcctcctcctcctcgctctcgtggtcatcgtacaccactttgttgacggccctccgggccgcggtggtccgggccaggtggccgccgccgcccccgccccccgtcctgccgcccccgcctcctcgccccccccggcccggggcgctggtgctggggggggccggcggcggcggcggcggcttcctccggctactgctgccccccctgggcgagctcagccgcgtcttgggcgccacctcagcctgggcggcggcccacctgccccggctgctgccgcggtgccgcgagcggagccccccgatgggtccggacgtgggcggcggcggcggtggcggcggggccggggcgcagcgctccgcagcgggagccgcgggctgcttgggcggcctgccccgccggcccctcatgtcggagccgaggcggggggagaaggaaagcgaagggggaggggcgggcgcagggggggcggtggggagcgccggggccgggtggggaggcccgcggggccgggcgggaggggcccggccgacggaagcgggtggagggagaaggctcaatccgaattgctggggccccactccggatcgccttcagccgccatcttgtttcttccct

SEQ ID NO: 9366 - RNA, 8800 nt, Homo sapiens
  source 1..8800: mol_type = other RNA
aggaagccctggaggggctggaggagctggtgtcactggggggcagggtgcagctactgctgtggcctgagccaactgcatcaggtctttttctttcttaattttcaggtctctcttcagctcttcctgcacttcaatttgcagatccttgtccaggagtgctctcttcttcaggatctcggctctgagctgctctttgtgcttgaagagcagagctgacagcttagtggcattctgcttgctacgtttctgctccacactctcttcacgcttccgtttttttgctgcctgtttttcttctttatctatcttatccaaaatatacttcatcacctggttacagacaatcattctttgattctcttctctttcagctggagtcatgctctttttctgttttaaatgttctattacagcattatgcttcatcaccacctgtttctgaatgatttcactttgattagaagcttggagggtgtgttcacgcttaatttctatctgttgctgtttcttcttttgctgctgatccctgagttgctgaaccctttgcaactgctcttgcacactggctgcctgcactgtaaccacattctgaatctggtgagtctgcacagcactgctttgctgaatttggataggtaactggagtttgatttgctggggcacaccactttgctgagcctgtatctgagccacaacctgtgactggatctgagagagaacctggacttgttgttgcagctgaggcacagcaatgacttggggctgtggctgctgtatttgtagctgaggacgggatggggatgaaacagtaacttgatttaaagtttgtcctgatgaaagagtttgagttgaagactgtacctggggttgtgactgtggctggccttgggaaggtatctgaagagatgtatgtggttgaattggaatcggttgtgaggttgtagtctgaacctgggattgttgtccaggagacagttgggatggagttgatggacgtattcgagtctgtgatggactttggacacgaacaggagactgtccttggacattactttgaggctgagactgtgctgcaacttggggcttggatgactgtgcgtgggtgggttgtgcttcagaagggacatgggatgaaacagttgtttgggtctgaacttcaggctgagtctgaacttcaggctgagctggggactggggctgggtttggggctggggctgagctgaaggctgagcagtctgtggctgggcttctgctggacccacacttgatgactgagctggtggcagggttttgtcttgatgtacctgcatctggggtgacagtttactctgcctttgttcacctgtacctgctgctgtcgtggaaacagtggtggtggtggtgctggctgtggtggctgttgttgccaatggggtaaagaggaatcgctgaacagtaccatttggcattgcagcttgcattagctgctggcctgggcctgggagtacagtcaccccttgaggtatcaactgcaactgtccagtagtttgaccttgtccttgaattactactgtcaaaccttgattgccaccgtggccctgtgttaactgagtaagttgagccatggtgagcttcacttgtccttgttgggggcgagggggttgtgaggctgaagactgtatatttgaagtggacgttgctgaagttaagcttttctgcccaggtgttgaggaaaccgtgttaggggcggagactgcagtggagacaggctgccccctgatgatttgagtcatcacttgctgaggagcacctggctgtaccatcacaggtgttcgaataattgcctttcctagtgttgactgttggagtggtgttctaatcacggtcataccagggcgaatctgaggccctgtgattacttgtgaattgcttgtggttcctccagagcctgaggtattgggcctaattgtgactgttgctgtcctgggctggaatgaagtaaaggtttgctgactggtacctgtacttgatggaatgatacccaggactttctgctgtacttgaacaacgcctccttgtgttgctggcacatttacagcgacaatcttgctgtttgcaggaagtggcagtttggtaattacttttcctgccatagtgactggattgcctgtaatttggaacgtctgacctgtgctggcaatggttgtagcagatgtggcagctgtgctggtggctgaatttgactggccttgcttaacccatgtagcaaaggtttgatgaaagttcttgttttgttggaatgttactgtagctggagatccaactttagtagttagtaccattttggttccagttgtaactgagccacttatgggggccaccataaccttctgtgctggagagatggtgctggttgtactgcttgttggggaagtagtggaagttgcaatcactgtcggcttctgctgctccagtcgtttcttagcctgttgctcaactgcttgtgccttttctttctccactctctcagcaaatgccctgatctcccacaattccagttcttcttctgctacccaggtttcaataataacagggccagtttgcttgggcgtttctggtctctttggccgcagtgcacttgatcgaaggcctttcctctgaggtgtaggcgtttcttttggtgtttctggaactccaatgggacaaatgattttcctgatacaatattcagatcgaatgccataaggaccaacatctctcctcttaattatttctgttgttgtgatttcagtttcggatgtttctgtccgtgtagtccctcctcctggaggagccttggccgccatatcatcccatctcaaacttgcccacagtaaccgtaacatcaggctcactccagctaaggactttactgtctgaagtctatacctccaagtgatgccaaaggtcggtctaggagaaggatatggccatatatccaaagcaggttttgcattgtaattaaaataagggacctctcggattcctccttttcgggccaacttttttaagtcatcattaggcaaaacaaaaatgctcttcttgctgctcttggtaacaaattttctataggatggcagagctgtacctgaacgagtcttctttggtcttgaaaatttcatcagtttcactttgtctcgtgtggaatactctttgctcacagtcatagatgtaaccagtgtgcctcccgtggtggtcagggagtctgtcactgtcgtggtgaccacggttttgctctgctcctttacagagatgatgtccacactgccgcctgtggagggtgtggaaagcttggtcactgttgtagtggtggttgtgacagtggattttgcacaattttctgtggaagaaaccacagtttgcttatcgcctttttctaccttgatcacagtttttgattctgtggccactgtggaggtcatcgtggtgacttctgtgatgacggtttttcttttagattctccattgacattttcatttttgttgatgggcagaccattttcatcaataaagtcattactgagattagattcctcttcagaagtaataggtgatgaagtaactttcttaacttctgaggtttctatttccatatcttctacctgattaactgaattgctttctggacaagatgctgagggtgtggtcgtctgtgtactgtcagactctttggttgatggcagggtctcaaggctatctcggtagttaccttcagcatctgaagaactcagcaaatgcgattttgtttcggagctgtttctttcattaaaatcttccatgatgacatcaccattaatgaatggccttatagcagattctttaacagtcaatgatttaatatcattctcagggattattttatttatattattaacctttggttcaacattaccacttactactctactctcagaaatttctttcaagcattcacctttcaaatatattttgggtttattatcttttccatttatttgaaatgtacttgttctctgtcctttcttttcagactctcgattttcattattctttttgtcagtggtattttttagctttatttgatcactacatttattaactggtctctcctctaatttcttctgctgacttggttttttaccatttgcttcagtccccttgaccggcagcctgtcctcacagtttccagtggactcaccagaaaccaactcacactttaacggctccaagacttcaacatcttgttctcgagttctgaactgttcagaaatgctttcattgctattctgaacaatcatatcttcttcactgctatcctgaatagacacggtatcagaactattttccaaagtgctattagattcagagtcacatcccagttttccttcaaagtccattgctcttgacagaggtgtggcatctctgtcattggtacttttaggcactgatgaatgtaaagcactcttggaagaagaaacaatggtgtcactttcctcctgtatgagcggttttttgttcttacagatcaaagtaccaatatcatctgcactggctagtttagagtcatcgatgaaaaaatcatttccttttgttttactcttactgggttcctggcctctactggcaaggtcagagactttttcttctatgtcattttcaatggaattttgtttcggacattttgtttctgggctccgaatggagacatcatctaacactcgatcttttggataaagtttgtttgtggtatgactaggatcactcattctaagaactgaggaatcactttctgaacatccctgaatcaagtcctcaggttgatcattatttgcatttgggctctgttcttgtctcatcgagtcactctgacacccttcttttgctttcgttattactggtgattcagagagattttttgaagaatttgtagaagtctttcctatacccttaattccaccctccaacttgattttttcgagtcgctgtttttcttccagtgtaaactgtttaattctcctttcaagaagtccatctagtttggatgattttgttttctttttgtaactagtccttagatgaaaaccctcactaacattgaccacatctacttgagaactctcctgacaatttacatgtgactctgttttcatgtcatcgtctacttccattggttcttccttgcagggtttatcactgtcagaatctaagagctccttcacatcttggtccttcttctcagtaatctttgagatatccatttcattttggtctgctccttttgcagcatctgaaccttttacctcatctttttcagaatcaggctctatttttattttttttggacttcgtgaacattttcttttatctgactcatccatattttcatccatattatttttggttccttctaacgactttctgtaattcacattagtattgcctggcaatttaggaacaaacctataaacatgagttttactaatccagctccaaccaccatatcctgtcactctgtactcttcacctttttgtttccaaacctgatgcttaactggaaatgtgtattttacccatgtcgcttgctgcatcgtttcttcttcttcctgtttcttctctttttttttgactttctccttttcttctctttcaattgatgtcatccggtgtaacctggtatgtcctaaagattctcgccatattggtagcatcacaactggtttaactgcacactccaaaatggctaaagccaatgcaaattctctgggtttgctacacatctgaactgccttgatccaatttgccctatgtgatgcccagttgggatgaagaaaggatgaagggatgttgttttctaattgggtgatagtcagtctcagagtagatatggtaagaactttggacccatggacagaaccgttccatttgaactctcctgctggagtcagacagaacttatgtgcaagatgccttctcttatcatggtcttctctgtgctggtgcttattcaaagcaaatgaattggtggagtattgattgtggtagacgcgatacttcccttcttgacccaatttaaaataattgttgatatttcctttcatgatcacttcctttttggtgctcaaccgtgaaatttctccttgagagttaactaccagtacctctttgccctccttaaataatttatttgcttcatgtgcagcggctgccacctgctggctcttcagctgactaagtttgctatctggattccgcaatctggtgatgattcgagttgagccagatgctccttttccagctccaggagattcacttagctccccgttggacttctccgatttgaaatcacctactatctcttcctgaatagagacaggtgtatgagattctctttctccattttcaggatcatcagctgccttagcagattcactctgggaagaatttagttcactgctgctgttactgttttccagattaggctggatggaggtagtggtagcactagtgttactgctctcacatgtcttgttaggttcttctggcacatcctgggggagctcagatgccaccttcttctctgccatgttgctgctatcgggggtttctgagagacaccccacagggctcctcccttcagagggactagtctcttctgaagttgcatttgttgtgttgtcgccaagatttgctgacacagagttacctttatccccaacttctgttggctcctcagattttccttgctcagggtcatcatctggtgttttgtcgtcactgtctttttcaagggactggtcttcaaattcttctctgtttttctcagcatctttagagtcattctcagtctcattcttgtctttttctgtttcttctgggcttttaacattatcaatgtctccctttttggctcttatggattccaaaatttcttcattagctgccgccagaaaggatttgttactgccccgagccttattggtcaggtcttcagttatgtccatgtgtcggtggatttcttcacgcatttcttctagaattttgcagagttctgcttcccaataatctttgtctagacagtcaattaattctgcaagttggacctttgtgctgtaataccaaattttcttttcattttcattttctgtatcttcttctattatgagtcttcggttcaagaaccagtatttcctccgacttctatcatatccaataggttcatgtcgaatatatggtttatttttttggatttcagcaacacagtcagtcacaccaggcaccttgtgtgctacacagacttcacactgccactcgtcctctggcacctcctcaagaggtggcttcacacattccaaatggtatactgctgaacatgtctcacagcaaagcaaatccccaagtttgtgacaaaccctacaatggtcatcatactgtatcaccccttcagacatcaattcctctcgagcaatatttgttgtaagaaactgatcgactagaaactgtagaactttgatcttgttctctactggtccatatgggtagtcctctgcctcttggtaaggaagaacgtgatggtactccttatcactctcacagtacacccgcagcacctctggccacgtcatcccatctatgaaatacagtgtggaattaacgctatctttcagatcagcaggtccaaaggtagtattggaagtgtcttcttcacgcagaactgctttcaaaagcacaacatgcatctctgccatgagtgtgcactgctcttggctcaccagagctgcacaaaagtcctcaaagcgaaaaggagataatctcaaaacagtgccaaagttccgcagtacctcgtaaatggcaatgacattcattatatgctcattaggcaccattaaatcctcagaggacttgggaaattcaaggggcgggatgtctttttcttccaatataggagaacgaggccgatgtactcttggttttcgcctacctggagtgctgctgtaggtactatggctcctgaagctgctttccgtgcagtaactggcgtcgtcgtcgtcgtcttccatctcctccggataatcggagtcatcgtcgtcctcttccatctcatcctcctcgtcgtcctcagaatcctgggtctcctcggcgtcgccgtcctcctcctcctcctcctcggagaccatgtcctcctcttcctcctcctcctcgctctcgtggtcatcgtacaccactttgttgacggccctccgggccgcggtggtccgggccaggtggccgccgccgcccccgccccccgtcctgccgcccccgcctcctcgccccccccggcccggggcgctggtgctggggggggccggcggcggcggcggcggcttcctccggctactgctgccccccctgggcgagctcagccgcgtcttgggcgccacctcagcctgggcggcggcccacctgccccggctgctgccgcggtgccgcgagcggagccccccgatgggtccggacgtgggcggcggcggcggtggcggcggggccggggcgcagcgctccgcagcgggagccgcgggctgcttgggcggcctgccccgccggcccctcatgtcggagccgaggcggggggagaaggaaagcgaagggggaggggcgggcgcagggggggcggtggggagcgccggggccgggtggggaggcccgcggggccgggcgggaggggcccggccgacggaagcgggtggagggagaaggctcaatccgaattgctggggccccactccggatcgccttcagccgccatcttgtttcttccct

SEQ ID NO: 9367 - RNA, 8611 nt, Homo sapiens
  source 1..8611: mol_type = other RNA
aggaagccctggaggggctggaggagctggtgtcactggggggcagggtgcagctactgctgtggcctgagccaactgcatcaggtctttttctttcttaattttcaggtctctcttcagctcttcctgcacttcaatttgcagatccttgtccaggagtgctctcttcttcaggatctcggctctgagctgctctttgtgcttgaagagcagagctgacagcttagtggcattctgcttgctacgtttctgctccacactctcttcacgcttccgtttttttgctgcctgtttttcttctttatctatcttatccaaaatatacttcatcacctggttacagacaatcattctttgattctcttctctttcagctggagtcatgctctttttctgttttaaatgttctattacagcattatgcttcatcaccacctgtttctgaatgatttcactttgattagaagcttggagggtgtgttcacgcttaatttctatctgttgctgtttcttcttttgctgctgatccctgagttgctgaaccctttgcaactgctcttgcacactggctgcctgcactgtaaccacattctgaatctggtgagtctgcacagcactgctttgctgaatttggataggtaactggagtttgatttgctggggcacaccactttgctgagcctgtatctgagccacaacctgtgactggatctgagagagaacctggacttgttgttgcagctgaggcacagcaatgacttggggctgtggctgctgtatttgtagctgaggacgggatggggatgaaacagtaacttgatttaaagtttgtcctgatgaaagagtttgagttgaagactgtacctggggttgtgactgtggctggccttgggaaggtatctgaagagatgtatgtggttgaattggaatcggttgtgaggttgtagtctgaacctgggattgttgtccaggagacagttgggatggagttgatggacgtattcgagtctgtgatggactttggacacgaacaggagactgtccttggacattactttgaggctgagactgtgctgcaacttggggcttggatgactgtgcgtgggtgggttgtgcttcagaagggacatgggatgaaacagttgtttgggtctgaacttcaggctgagtctgaacttcaggctgagctggggactggggctgggtttggggctggggctgagctgaaggctgagcagtctgtggctgggcttctgctggacccacacttgatgactgagctggtggcagggttttgtcttgatgtacctgcatctggggtgacagtttactctgcctttgttcacctgtacctgctgctgtcgtggaaacagtggtggtggtggtgctggctgtggtggctgttgttgccaatggggtaaagaggaatcgctgaacagtaccatttggcattgcagcttgcattagctgctggcctgggcctgggagtacagtcaccccttgaggtatcaactgcaactgtccagtagtttgaccttgtccttgaattactactgtcaaaccttgattgccaccgtggccctgtgttaactgagtaagttgagccatggtgagcttcacttgtccttgttgggggcgagggggttgtgaggctgaagactgtatatttgaagtggacgttgctgaagttaagcttttctgcccaggtgttgaggaaaccgtgttaggggcggagactgcagtggagacaggctgccccctgatgatttgagtcatcacttgctgaggagcacctggctgtaccatcacaggtgttcgaataattgcctttcctagtgttgactgttggagtggtgttctaatcacggtcataccagggcgaatctgaggccctgtgattacttgtgaattgcttgtggttcctccagagcctgaggtattgggcctaattgtgactgttgctgtcctgggctggaatgaagtaaaggtttgctgactggtacctgtacttgatggaatgatacccaggactttctgctgtacttgaacaacgcctccttgtgttgctggcacatttacagcgacaatcttgctgtttgcaggaagtggcagtttggtaattacttttcctgccatagtgactggattgcctgtaatttggaacgtctgacctgtgctggcaatggttgtagcagatgtggcagctgtgctggtggctgaatttgactggccttgcttaacccatgtagcaaaggtttgatgaaagttcttgttttgttggaatgttactgtagctggagatccaactttagtagttagtaccattttggttccagttgtaactgagccacttatgggggccaccataaccttctgtgctggagagatggtgctggttgtactgcttgttggggaagtagtggaagttgcaatcactgtcggcttctgctgctccagtcgtttcttagcctgttgctcaactgcttgtgccttttctttctccactctctcagcaaatgccctgatctcccacaattccagttcttcttctgctacccaggtttcaataataacagggccagtttgcttgggcgtttctggtctctttggccgcagtgcacttgatcgaaggcctttcctctgaggtgtaggcgtttcttttggtgtttctggaactccaatgggacaaatgattttcctgatacaatattcagatcgaatgccataaggaccaacatctctcctcttaattatttctgttgttgtgatttcagtttcggatgtttctgtccgtgtagtccctcctcctggaggagccttggccgccatatcatcccatctcaaacttgcccacagtaaccgtaacatcaggctcactccagctaaggactttactgtctgaagtctatacctccaagtgatgccaaaggtcggtctaggagaaggatatggccatatatccaaagcaggttttgcattgtaattaaaataagggacctctcggattcctccttttcgggccaacttttttaagtcatcattaggcaaaacaaaaatgctcttcttgctgctcttggtaacaaattttctataggatggcagagctgtacctgaacgagtcttctttggtcttgaaaatttcatcagtttcactttgtctcgtgtggaatactctttgctcacagtcatagatgtaaccagtgtgcctcccgtggtggtcagggagtctgtcactgtcgtggtgaccacggttttgctctgctcctttacagagatgatgtccacactgccgcctgtggagggtgtggaaagcttggtcactgttgtagtggtggttgtgacagtggattttgcacaattttctgtggaagaaaccacagtttgcttatcgcctttttctaccttgatcacagtttttgattctgtggccactgtggaggtcatcgtggtgacttctgtgatgacggtttttcttttagattctccattgacattttcatttttgttgatgggcagaccattttcatcaataaagtcattactgagattagattcctcttcagaagtaataggtgatgaagtaactttcttaacttctgaggtttctatttccatatcttctacctgattaactgaattgctttctggacaagatgctgagggtgtggtcgtctgtgtactgtcagactctttggttgatggcagggtctcaaggctatctcggtagttaccttcagcatctgaagaactcagcaaatgcgattttgtttcggagctgtttctttcattaaaatcttccatgatgacatcaccattaatgaatggccttatagcagattctttaacagtcaatgatttaatatcattctcagggattattttatttatattattaacctttggttcaacattaccacttactactctactctcagaaatttctttcaagcattcacctttcaaatatattttgggtttattatcttttccatttatttgaaatgtacttgttctctgtcctttcttttcagactctcgattttcattattctttttgtcagtggtattttttagctttatttgatcactacatttattaactggtctctcctctaatttcttctgctgacttggttttttaccatttgcttcagtccccttgaccggcagcctgtcctcacagtttccagtggactcaccagaaaccaactcacactttaacggctccaagacttcaacatcttgttctcgagttctgaactgttcagaaatgctttcattgctattctgaacaatcatatcttcttcactgctatcctgaatagacacggtatcagaactattttccaaagtgctattagattcagagtcacatcccagttttccttcaaagtccattgctcttgacagaggtgtggcatctctgtcattggtacttttaggcactgatgaatgtaaagcactcttggaagaagaaacaatggtgtcactttcctcctgtatgagcggttttttgttcttacagatcaaagtaccaatatcatctgcactggctagtttagagtcatcgatgaaaaaatcatttccttttgttttactcttactgggttcctggcctctactggcaaggtcagagactttttcttctatgtcattttcaatggaattttgtttcggacattttgtttctgggctccgaatggagacatcatctaacactcgatcttttggataaagtttgtttgtggtatgactaggatcactcattctaagaactgaggaatcactttctgaacatccctgaatcaagtcctcaggttgatcattatttgcatttgggctctgttcttgtctcatcgagtcactctgacacccttcttttgctttcgttattactggtgattcagagagattttttgaagaatttgtagaagtctttcctatacccttaattccaccctccaacttgattttttcgagtcgctgtttttcttccagtgtaaactgtttaattctcctttcaagaagtccatctagtttggatgattttgttttctttttgtaactagtccttagatgaaaaccctcactaacattgaccacatctacttgagaactctcctgacaatttacatgtgactctgttttcatgtcatcgtctacttccattggttcttccttgcagggtttatcactgtcagaatctaagagctccttcacatcttggtccttcttctcagtaatctttgagatatccatttcattttggtctgctccttttgcagcatctgaaccttttacctcatctttttcagaatcaggctctatttttattttttttggacttcgtgaacattttcttttatctgactcatccatattttcatccatattatttttggttccttctaacgactttctgtaattcacattagtattgcctggcaatttaggaacaaacctataaacatgagttttactaatccagctccaaccaccatatcctgtcactctgtactcttcacctttttgtttccaaacctgatgcttaactggaaatgtgtattttacccatgtcgcttgctgcatcgtttcttcttcttcctgtttcttctctttttttttgactttctccttttcttctctttcaattgatgtcatccggtgtaacctggtatgtcctaaagattctcgccatattggtagcatcacaactggtttaactgcacactccaaaatggctaaagccaatgcaaattctctgggtttgctacacatctgaactgccttgatccaatttgccctatgtgatgcccagttgggatgaagaaaggatgaagggatgttgttttctaattgggtgatagtcagtctcagagtagatatggtaagaactttggacccatggacagaaccgttccatttgaactctcctgctggagtcagacagaacttatgtgcaagatgccttctcttatcatggtcttctctgtgctggtgcttattcaaagcaaatgaattggtggagtattgattgtggtagacgcgatacttcccttcttgacccaatttaaaataattgttgatatttcctttcatgatcacttcctttttggtgctcaaccgtgaaatttctccttgagagttaactaccagtacctctttgccctccttaaataatttatttgcttcatgtgcagcggctgccacctgctggctcttcagctgactaagtttgctatctggattccgcaatctggtgatgattcgagttgagccagatgctccttttccagctccaggagattcacttagctccccgttggacttctccgatttgaaatcacctactggcacatcctgggggagctcagatgccaccttcttctctgccatgttgctgctatcgggggtttctgagagacaccccacagggctcctcccttcagagggactagtctcttctgaagttgcatttgttgtgttgtcgccaagatttgctgacacagagttacctttatccccaacttctgttggctcctcagattttccttgctcagggtcatcatctggtgttttgtcgtcactgtctttttcaagggactggtcttcaaattcttctctgtttttctcagcatctttagagtcattctcagtctcattcttgtctttttctgtttcttctgggcttttaacattatcaatgtctccctttttggctcttatggattccaaaatttcttcattagctgccgccagaaaggatttgttactgccccgagccttattggtcaggtcttcagttatgtccatgtgtcggtggatttcttcacgcatttcttctagaattttgcagagttctgcttcccaataatctttgtctagacagtcaattaattctgcaagttggacctttgtgctgtaataccaaattttcttttcattttcattttctgtatcttcttctattatgagtcttcggttcaagaaccagtatttcctccgacttctatcatatccaataggttcatgtcgaatatatggtttatttttttggatttcagcaacacagtcagtcacaccaggcaccttgtgtgctacacagacttcacactgccactcgtcctctggcacctcctcaagaggtggcttcacacattccaaatggtatactgctgaacatgtctcacagcaaagcaaatccccaagtttgtgacaaaccctacaatggtcatcatactgtatcaccccttcagacatcaattcctctcgagcaatatttgttgtaagaaactgatcgactagaaactgtagaactttgatcttgttctctactggtccatatgggtagtcctctgcctcttggtaaggaagaacgtgatggtactccttatcactctcacagtacacccgcagcacctctggccacgtcatcccatctatgaaatacagtgtggaattaacgctatctttcagatcagcaggtccaaaggtagtattggaagtgtcttcttcacgcagaactgctttcaaaagcacaacatgcatctctgccatgagtgtgcactgctcttggctcaccagagctgcacaaaagtcctcaaagcgaaaaggagataatctcaaaacagtgccaaagttccgcagtacctcgtaaatggcaatgacattcattatatgctcattaggcaccattaaatcctcagaggacttgggaaattcaaggggcgggatgtctttttcttccaatataggagaacgaggccgatgtactcttggttttcgcctacctggagtgctgctgtaggtactatggctcctgaagctgctttccgtgcagtaactggcgtcgtcgtcgtcgtcttccatctcctccggataatcggagtcatcgtcgtcctcttccatctcatcctcctcgtcgtcctcagaatcctgggtctcctcggcgtcgccgtcctcctcctcctcctcctcggagaccatgtcctcctcttcctcctcctcctcgctctcgtggtcatcgtacaccactttgttgacggccctccgggccgcggtggtccgggccaggtggccgccgccgcccccgccccccgtcctgccgcccccgcctcctcgccccccccggcccggggcgctggtgctggggggggccggcggcggcggcggcggcttcctccggctactgctgccccccctgggcgagctcagccgcgtcttgggcgccacctcagcctgggcggcggcccacctgccccggctgctgccgcggtgccgcgagcggagccccccgatgggtccggacgtgggcggcggcggcggtggcggcggggccggggcgcagcgctccgcagcgggagccgcgggctgcttgggcggcctgccccgccggcccctcatgtcggagccgaggcggggggagaaggaaagcgaagggggaggggcgggcgcagggggggcggtggggagcgccggggccgggtggggaggcccgcggggccgggcgggaggggcccggccgacggaagcgggtggagggagaaggctcaatccgaattgctggggccccactccggatcgccttcagccgccatcttgtttcttccct

SEQ ID NO: 9368 - RNA, 8608 nt, Homo sapiens
  source 1..8608: mol_type = other RNA
aggaagccctggaggggctggaggagctggtgtcactggggggcagggtgcagctactgctgtggcctgagccaactgcatcaggtctttttctttcttaattttcaggtctctcttcagctcttcctgcacttcaatttgcagatccttgtccaggagtgctctcttcttcaggatctcggctctgagctgctctttgtgcttgaagagcagagctgacagcttagtggcattctgcttgctacgtttctgctccacactctcttcacgcttccgtttttttgctgcctgtttttcttctttatctatcttatccaaaatatacttcatcacctggttacagacaatcattctttgattctcttctctttcagctggagtcatgctctttttctgttttaaatgttctattacagcattatgcttcatcaccacctgtttctgaatgatttcactttgattagaagcttggagggtgtgttcacgcttaatttctatctgttgctgtttcttcttttgctgctgatccctgagttgctgaaccctttgcaactgctcttgcacactggctgcctgcactgtaaccacattctgaatctggtgagtctgcacagcactgctttgctgaatttggataggtaactggagtttgatttgctggggcacaccactttgctgagcctgtatctgagccacaacctgtgactggatctgagagagaacctggacttgttgttgcagctgaggcacagcaatgacttggggctgtggctgctgtatttgtagctgaggacgggatggggatgaaacagtaacttgatttaaagtttgtcctgatgaaagagtttgagttgaagactgtacctggggttgtgactgtggctggccttgggaaggtatctgaagagatgtatgtggttgaattggaatcggttgtgaggttgtagtctgaacctgggattgttgtccaggagacagttgggatggagttgatggacgtattcgagtctgtgatggactttggacacgaacaggagactgtccttggacattactttgaggctgagactgtgctgcaacttggggcttggatgactgtgcgtgggtgggttgtgcttcagaagggacatgggatgaaacagttgtttgggtctgaacttcaggctgagtctgaacttcaggctgagctggggactggggctgggtttggggctggggctgagctgaaggctgagcagtctgtggctgggcttctgctggacccacacttgatgactgagctggtggcagggttttgtcttgatgtacctgcatctggggtgacagtttactctgcctttgttcacctgtacctgctgctgtcgtggaaacagtggtggtggtggtgctggctgtggtggctgttgttgccaatggggtaaagaggaatcgctgaacagtaccatttggcattgcagcttgcattagctgctggcctgggcctgggagtacagtcaccccttgaggtatcaactgcaactgtccagtagtttgaccttgtccttgaattactactgtcaaaccttgattgccaccgtggccctgtgttaactgagtaagttgagccatggtgagcttcacttgtccttgttgggggcgagggggttgtgaggctgaagactgtatatttgaagtggacgttgctgaagttaagcttttctgcccaggtgttgaggaaaccgtgttaggggcggagactgcagtggagacaggctgccccctgatgatttgagtcatcacttgctgaggagcacctggctgtaccatcacaggtgttcgaataattgcctttcctagtgttgactgttggagtggtgttctaatcacggtcataccagggcgaatctgaggccctgtgattacttgtgaattgcttgtggttcctccagagcctgaggtattgggcctaattgtgactgttgctgtcctgggctggaatgaagtaaaggtttgctgactggtacctgtacttgatggaatgatacccaggactttctgctgtacttgaacaacgcctccttgtgttgctggcacatttacagcgacaatcttgctgtttgcaggaagtggcagtttggtaattacttttcctgccatagtgactggattgcctgtaatttggaacgtctgacctgtgctggcaatggttgtagcagatgtggcagctgtgctggtggctgaatttgactggccttgcttaacccatgtagcaaaggtttgatgaaagttcttgttttgttggaatgttactgtagctggagatccaactttagtagttagtaccattttggttccagttgtaactgagccacttatgggggccaccataaccttctgtgctggagagatggtgctggttgtactgcttgttggggaagtagtggaagttgcaatcactgtcggcttctgctgctccagtcgtttcttagcctgttgctcaactgcttgtgccttttctttctccactctctcagcaaatgccctgatctcccacaattccagttcttcttctgctacccaggtttcaataataacagggccagtttgcttgggcgtttctggtctctttggccgcagtgcacttgatcgaaggcctttcctctgaggtgtaggcgtttcttttggtgtttctggaactccaatgggacaaatgattttcctgatacaatattcagatcgaatgccataaggaccaacatctctcctcttaattatttctgttgttgtgatttcagtttcggatgtttctgtccgtgtagtccctcctcctggaggagccttggccgccatatcatcccatctcaaacttgcccacagtaaccgtaacatcaggctcactccagctaaggactttactgtctgaagtctatacctccaagtgatgccaaaggtcggtctaggagaaggatatggccatatatccaaagcaggttttgcattgtaattaaaataagggacctctcggattcctccttttcgggccaacttttttaagtcatcattaggcaaaacaaaaatgctcttcttgctgctcttggtaacaaattttctataggatggcagagctgtacctgaacgagtcttctttggtcttgaaaatttcatcagtttcactttgtctcgtgtggaatactctttgctcacagtcatagatgtaaccagtgtgcctcccgtggtggtcagggagtctgtcactgtcgtggtgaccacggttttgctctgctcctttacagagatgatgtccacactgccgcctgtggagggtgtggaaagcttggtcactgttgtagtggtggttgtgacagtggattttgcacaattttctgtggaagaaaccacagtttgcttatcgcctttttctaccttgatcacagtttttgattctgtggccactgtggaggtcatcgtggtgacttctgtgatgacggtttttcttttagattctccattgacattttcatttttgttgatgggcagaccattttcatcaataaagtcattactgagattagattcctcttcagaagtaataggtgatgaagtaactttcttaacttctgaggtttctatttccatatcttctacctgattaactgaattgctttctggacaagatgctgagggtgtggtcgtctgtgtactgtcagactctttggttgatggcagggtctcaaggctatctcggtagttaccttcagcatctgaagaactcagcaaatgcgattttgtttcggagctgtttctttcattaaaatcttccatgatgacatcaccattaatgaatggccttatagcagattctttaacagtcaatgatttaatatcattctcagggattattttatttatattattaacctttggttcaacattaccacttactactctactctcagaaatttctttcaagcattcacctttcaaatatattttgggtttattatcttttccatttatttgaaatgtacttgttctctgtcctttcttttcagactctcgattttcattattctttttgtcagtggtattttttagctttatttgatcactacatttattaactggtctctcctctaatttcttctgctgacttggttttttaccatttgcttcagtccccttgaccggcagcctgtcctcacagtttccagtggactcaccagaaaccaactcacactttaacggctccaagacttcaacatcttgttctcgagttctgaactgttcagaaatgctttcattgctattctgaacaatcatatcttcttcactgctatcctgaatagacacggtatcagaactattttccaaagtgctattagattcagagtcacatcccagttttccttcaaagtccattgctcttgacagaggtgtggcatctctgtcattggtacttttaggcactgatgaatgtaaagcactcttggaagaagaaacaatggtgtcactttcctcctgtatgagcggttttttgttcttacagatcaaagtaccaatatcatctgcactggctagtttagagtcatcgatgaaaaaatcatttccttttgttttactcttactgggttcctggcctctactggcaaggtcagagactttttcttctatgtcattttcaatggaattttgtttcggacattttgtttctgggctccgaatggagacatcatctaacactcgatcttttggataaagtttgtttgtggtatgactaggatcactcattctaagaactgaggaatcactttctgaacatccctgaatcaagtcctcaggttgatcattatttgcatttgggctctgttcttgtctcatcgagtcactctgacacccttcttttgctttcgttattactggtgattcagagagattttttgaagaatttgtagaagtctttcctatacccttaattccaccctccaacttgattttttcgagtcgctgtttttcttccagtgtaaactgtttaattctcctttcaagaagtccatctagtttggatgattttgttttctttttgtaactagtccttagatgaaaaccctcactaacattgaccacatctacttgagaactctcctgacaatttacatgtgactctgttttcatgtcatcgtctacttccattggttcttccttgcagggtttatcactgtcagaatctaagagctccttcacatcttggtccttcttctcagtaatctttgagatatccatttcattttggtctgctccttttgcagcatctgaaccttttacctcatctttttcagaatcaggctctatttttattttttttggacttcgtgaacattttcttttatctgactcatccatattttcatccatattatttttggttccttctaacgactttctgtaattcacattagtattgcctggcaatttaggaacaaacctataaacatgagttttactaatccagctccaaccaccatatcctgtcactctgtactcttcacctttttgtttccaaacctgatgcttaactggaaatgtgtattttacccatgtcgcttgctgcatcgtttcttcttcttcctgtttcttctctttttttttgactttctccttttcttctctttcaattgatgtcatccggtgtaacctggtatgtcctaaagattctcgccatattggtagcatcacaactggtttaactgcacactccaaaatggctaaagccaatgcaaattctctgggtttgctacacatctgaactgccttgatccaatttgccctatgtgatgcccagttgggatgaagaaaggatgaagggatgttgttttctaattgggtgatagtcagtctcagagtagatatggtaagaactttggacccatggacagaaccgttccatttgaactctcctgctggagtcagacagaacttatgtgcaagatgccttctcttatcatggtcttctctgtgctggtgcttattcaaagcaaatgaattggtggagtattgattgtggtagacgcgatacttcccttcttgacccaatttaaaataattgttgatatttcctttcatgatcacttcctttttggtgctcaaccgtgaaatttctccttgagagttaactaccagtacctctttgccctccttaaataatttatttgcttcatgtgcagcggctgccacctgctggctcttcagctgactaagtttgctatctggattccgcaatctggtgatgattcgagttgagccagatgctccttttccagctccaggagattcacttagctccccgttggacttctccgatttgaaatcacctatctcttcctgaatagagacaggtgtatgagattctctttctccattttcaggatcatcagctgccttagcagattcactctgggaagaatttagttcactgctgctgttactgttttccagattaggctggatggaggtagtggtagcactagtgttactgctctcacatgtcttgttaggttcttcctcagattttccttgctcagggtcatcatctggtgttttgtcgtcactgtctttttcaagggactggtcttcaaattcttctctgtttttctcagcatctttagagtcattctcagtctcattcttgtctttttctgtttcttctgggcttttaacattatcaatgtctccctttttggctcttatggattccaaaatttcttcattagctgccgccagaaaggatttgttactgccccgagccttattggtcaggtcttcagttatgtccatgtgtcggtggatttcttcacgcatttcttctagaattttgcagagttctgcttcccaataatctttgtctagacagtcaattaattctgcaagttggacctttgtgctgtaataccaaattttcttttcattttcattttctgtatcttcttctattatgagtcttcggttcaagaaccagtatttcctccgacttctatcatatccaataggttcatgtcgaatatatggtttatttttttggatttcagcaacacagtcagtcacaccaggcaccttgtgtgctacacagacttcacactgccactcgtcctctggcacctcctcaagaggtggcttcacacattccaaatggtatactgctgaacatgtctcacagcaaagcaaatccccaagtttgtgacaaaccctacaatggtcatcatactgtatcaccccttcagacatcaattcctctcgagcaatatttgttgtaagaaactgatcgactagaaactgtagaactttgatcttgttctctactggtccatatgggtagtcctctgcctcttggtaaggaagaacgtgatggtactccttatcactctcacagtacacccgcagcacctctggccacgtcatcccatctatgaaatacagtgtggaattaacgctatctttcagatcagcaggtccaaaggtagtattggaagtgtcttcttcacgcagaactgctttcaaaagcacaacatgcatctctgccatgagtgtgcactgctcttggctcaccagagctgcacaaaagtcctcaaagcgaaaaggagataatctcaaaacagtgccaaagttccgcagtacctcgtaaatggcaatgacattcattatatgctcattaggcaccattaaatcctcagaggacttgggaaattcaaggggcgggatgtctttttcttccaatataggagaacgaggccgatgtactcttggttttcgcctacctggagtgctgctgtaggtactatggctcctgaagctgctttccgtgcagtaactggcgtcgtcgtcgtcgtcttccatctcctccggataatcggagtcatcgtcgtcctcttccatctcatcctcctcgtcgtcctcagaatcctgggtctcctcggcgtcgccgtcctcctcctcctcctcctcggagaccatgtcctcctcttcctcctcctcctcgctctcgtggtcatcgtacaccactttgttgacggccctccgggccgcggtggtccgggccaggtggccgccgccgcccccgccccccgtcctgccgcccccgcctcctcgccccccccggcccggggcgctggtgctggggggggccggcggcggcggcggcggcttcctccggctactgctgccccccctgggcgagctcagccgcgtcttgggcgccacctcagcctgggcggcggcccacctgccccggctgctgccgcggtgccgcgagcggagccccccgatgggtccggacgtgggcggcggcggcggtggcggcggggccggggcgcagcgctccgcagcgggagccgcgggctgcttgggcggcctgccccgccggcccctcatgtcggagccgaggcggggggagaaggaaagcgaagggggaggggcgggcgcagggggggcggtggggagcgccggggccgggtggggaggcccgcggggccgggcgggaggggcccggccgacggaagcgggtggagggagaaggctcaatccgaattgctggggccccactccggatcgccttcagccgccatcttgtttcttccct

SEQ ID NO: 9369 - RNA, 8797 nt, Homo sapiens
  source 1..8797: mol_type = other RNA
aggaagccctggaggggctggaggagctggtgtcactggggggcagggtgcagctactgctgtggcctgagccaactgcatcaggtctttttctttcttaattttcaggtctctcttcagctcttcctgcacttcaatttgcagatccttgtccaggagtgctctcttcttcaggatctcggctctgagctgctctttgtgcttgaagagcagagctgacagcttagtggcattctgcttgctacgtttctgctccacactctcttcacgcttccgtttttttgctgcctgtttttcttctttatctatcttatccaaaatatacttcatcacctggttacagacaatcattctttgattctcttctctttcagctggagtcatgctctttttctgttttaaatgttctattacagcattatgcttcatcaccacctgtttctgaatgatttcactttgattagaagcttggagggtgtgttcacgcttaatttctatctgttgctgtttcttcttttgctgctgatccctgagttgctgaaccctttgcaactgctcttgcacactggctgcctgcactgtaaccacattctgaatctggtgagtctgcacagcactgctttgctgaatttggataggtaactggagtttgatttgctggggcacaccactttgctgagcctgtatctgagccacaacctgtgactggatctgagagagaacctggacttgttgttgcagctgaggcacagcaatgacttggggctgtggctgctgtatttgtagctgaggacgggatggggatgaaacagtaacttgatttaaagtttgtcctgatgaaagagtttgagttgaagactgtacctggggttgtgactgtggctggccttgggaaggtatctgaagagatgtatgtggttgaattggaatcggttgtgaggttgtagtctgaacctgggattgttgtccaggagacagttgggatggagttgatggacgtattcgagtctgtgatggactttggacacgaacaggagactgtccttggacattactttgaggctgagactgtgctgcaacttggggcttggatgactgtgcgtgggtgggttgtgcttcagaagggacatgggatgaaacagttgtttgggtctgaacttcaggctgagtctgaacttcaggctgagctggggactggggctgggtttggggctggggctgagctgaaggctgagcagtctgtggctgggcttctgctggacccacacttgatgactgagctggtggcagggttttgtcttgatgtacctgcatctggggtgacagtttactctgcctttgttcacctgtacctgctgctgtcgtggaaacagtggtggtggtggtgctggctgtggtggctgttgttgccaatggggtaaagaggaatcgctgaacagtaccatttggcattgcagcttgcattagctgctggcctgggcctgggagtacagtcaccccttgaggtatcaactgcaactgtccagtagtttgaccttgtccttgaattactactgtcaaaccttgattgccaccgtggccctgtgttaactgagtaagttgagccatggtgagcttcacttgtccttgttgggggcgagggggttgtgaggctgaagactgtatatttgaagtggacgttgctgaagttaagcttttctgcccaggtgttgaggaaaccgtgttaggggcggagactgcagtggagacaggctgccccctgatgatttgagtcatcacttgctgaggagcacctggctgtaccatcacaggtgttcgaataattgcctttcctagtgttgactgttggagtggtgttctaatcacggtcataccagggcgaatctgaggccctgtgattacttgtgaattgcttgtggttcctccagagcctgaggtattgggcctaattgtgactgttgctgtcctgggctggaatgaagtaaaggtttgctgactggtacctgtacttgatggaatgatacccaggactttctgctgtacttgaacaacgcctccttgtgttgctggcacatttacagcgacaatcttgctgtttgcaggaagtggcagtttggtaattacttttcctgccatagtgactggattgcctgtaatttggaacgtctgacctgtgctggcaatggttgtagcagatgtggcagctgtgctggtggctgaatttgactggccttgcttaacccatgtagcaaaggtttgatgaaagttcttgttttgttggaatgttactgtagctggagatccaactttagtagttagtaccattttggttccagttgtaactgagccacttatgggggccaccataaccttctgtgctggagagatggtgctggttgtactgcttgttggggaagtagtggaagttgcaatcactgtcggcttctgctgctccagtcgtttcttagcctgttgctcaactgcttgtgccttttctttctccactctctcagcaaatgccctgatctcccacaattccagttcttcttctgctacccaggtttcaataataacagggccagtttgcttgggcgtttctggtctctttggccgcagtgcacttgatcgaaggcctttcctctgaggtgtaggcgtttcttttggtgtttctggaactccaatgggacaaatgattttcctgatacaatattcagatcgaatgccataaggaccaacatctctcctcttaattatttctgttgttgtgatttcagtttcggatgtttctgtccgtgtagtccctcctcctggaggagccttggccgccatatcatcccatctcaaacttgcccacagtaaccgtaacatcaggctcactccagctaaggactttactgtctgaagtctatacctccaagtgatgccaaaggtcggtctaggagaaggatatggccatatatccaaagcaggttttgcattgtaattaaaataagggacctctcggattcctccttttcgggccaacttttttaagtcatcattaggcaaaacaaaaatgctcttcttgctgctcttggtaacaaattttctataggatggcagagctgtacctgaacgagtcttctttggtcttgaaaatttcatcagtttcactttgtctcgtgtggaatactctttgctcacagtcatagatgtaaccagtgtgcctcccgtggtggtcagggagtctgtcactgtcgtggtgaccacggttttgctctgctcctttacagagatgatgtccacactgccgcctgtggagggtgtggaaagcttggtcactgttgtagtggtggttgtgacagtggattttgcacaattttctgtggaagaaaccacagtttgcttatcgcctttttctaccttgatcacagtttttgattctgtggccactgtggaggtcatcgtggtgacttctgtgatgacggtttttcttttagattctccattgacattttcatttttgttgatgggcagaccattttcatcaataaagtcattactgagattagattcctcttcagaagtaataggtgatgaagtaactttcttaacttctgaggtttctatttccatatcttctacctgattaactgaattgctttctggacaagatgctgagggtgtggtcgtctgtgtactgtcagactctttggttgatggcagggtctcaaggctatctcggtagttaccttcagcatctgaagaactcagcaaatgcgattttgtttcggagctgtttctttcattaaaatcttccatgatgacatcaccattaatgaatggccttatagcagattctttaacagtcaatgatttaatatcattctcagggattattttatttatattattaacctttggttcaacattaccacttactactctactctcagaaatttctttcaagcattcacctttcaaatatattttgggtttattatcttttccatttatttgaaatgtacttgttctctgtcctttcttttcagactctcgattttcattattctttttgtcagtggtattttttagctttatttgatcactacatttattaactggtctctcctctaatttcttctgctgacttggttttttaccatttgcttcagtccccttgaccggcagcctgtcctcacagtttccagtggactcaccagaaaccaactcacactttaacggctccaagacttcaacatcttgttctcgagttctgaactgttcagaaatgctttcattgctattctgaacaatcatatcttcttcactgctatcctgaatagacacggtatcagaactattttccaaagtgctattagattcagagtcacatcccagttttccttcaaagtccattgctcttgacagaggtgtggcatctctgtcattggtacttttaggcactgatgaatgtaaagcactcttggaagaagaaacaatggtgtcactttcctcctgtatgagcggttttttgttcttacagatcaaagtaccaatatcatctgcactggctagtttagagtcatcgatgaaaaaatcatttccttttgttttactcttactgggttcctggcctctactggcaaggtcagagactttttcttctatgtcattttcaatggaattttgtttcggacattttgtttctgggctccgaatggagacatcatctaacactcgatcttttggataaagtttgtttgtggtatgactaggatcactcattctaagaactgaggaatcactttctgaacatccctgaatcaagtcctcaggttgatcattatttgcatttgggctctgttcttgtctcatcgagtcactctgacacccttcttttgctttcgttattactggtgattcagagagattttttgaagaatttgtagaagtctttcctatacccttaattccaccctccaacttgattttttcgagtcgctgtttttcttccagtgtaaactgtttaattctcctttcaagaagtccatctagtttggatgattttgttttctttttgtaactagtccttagatgaaaaccctcactaacattgaccacatctacttgagaactctcctgacaatttacatgtgactctgttttcatgtcatcgtctacttccattggttcttccttgcagggtttatcactgtcagaatctaagagctccttcacatcttggtccttcttctcagtaatctttgagatatccatttcattttggtctgctccttttgcagcatctgaaccttttacctcatctttttcagaatcaggctctatttttattttttttggacttcgtgaacattttcttttatctgactcatccatattttcatccatattatttttggttccttctaacgactttctgtaattcacattagtattgcctggcaatttaggaacaaacctataaacatgagttttactaatccagctccaaccaccatatcctgtcactctgtactcttcacctttttgtttccaaacctgatgcttaactggaaatgtgtattttacccatgtcgcttgctgcatcgtttcttcttcttcctgtttcttctctttttttttgactttctccttttcttctctttcaattgatgtcatccggtgtaacctggtatgtcctaaagattctcgccatattggtagcatcacaactggtttaactgcacactccaaaatggctaaagccaatgcaaattctctgggtttgctacacatctgaactgccttgatccaatttgccctatgtgatgcccagttgggatgaagaaaggatgaagggatgttgttttctaattgggtgatagtcagtctcagagtagatatggtaagaactttggacccatggacagaaccgttccatttgaactctcctgctggagtcagacagaacttatgtgcaagatgccttctcttatcatggtcttctctgtgctggtgcttattcaaagcaaatgaattggtggagtattgattgtggtagacgcgatacttcccttcttgacccaatttaaaataattgttgatatttcctttcatgatcacttcctttttggtgctcaaccgtgaaatttctccttgagagttaactaccagtacctctttgccctccttaaataatttatttgcttcatgtgcagcggctgccacctgctggctcttcagctgactaagtttgctatctggattccgcaatctggtgatgattcgagttgagccagatgctccttttccagctccaggagattcacttagctccccgttggacttctccgatttgaaatcacctatctcttcctgaatagagacaggtgtatgagattctctttctccattttcaggatcatcagctgccttagcagattcactctgggaagaatttagttcactgctgctgttactgttttccagattaggctggatggaggtagtggtagcactagtgttactgctctcacatgtcttgttaggttcttctggcacatcctgggggagctcagatgccaccttcttctctgccatgttgctgctatcgggggtttctgagagacaccccacagggctcctcccttcagagggactagtctcttctgaagttgcatttgttgtgttgtcgccaagatttgctgacacagagttacctttatccccaacttctgttggctcctcagattttccttgctcagggtcatcatctggtgttttgtcgtcactgtctttttcaagggactggtcttcaaattcttctctgtttttctcagcatctttagagtcattctcagtctcattcttgtctttttctgtttcttctgggcttttaacattatcaatgtctccctttttggctcttatggattccaaaatttcttcattagctgccgccagaaaggatttgttactgccccgagccttattggtcaggtcttcagttatgtccatgtgtcggtggatttcttcacgcatttcttctagaattttgcagagttctgcttcccaataatctttgtctagacagtcaattaattctgcaagttggacctttgtgctgtaataccaaattttcttttcattttcattttctgtatcttcttctattatgagtcttcggttcaagaaccagtatttcctccgacttctatcatatccaataggttcatgtcgaatatatggtttatttttttggatttcagcaacacagtcagtcacaccaggcaccttgtgtgctacacagacttcacactgccactcgtcctctggcacctcctcaagaggtggcttcacacattccaaatggtatactgctgaacatgtctcacagcaaagcaaatccccaagtttgtgacaaaccctacaatggtcatcatactgtatcaccccttcagacatcaattcctctcgagcaatatttgttgtaagaaactgatcgactagaaactgtagaactttgatcttgttctctactggtccatatgggtagtcctctgcctcttggtaaggaagaacgtgatggtactccttatcactctcacagtacacccgcagcacctctggccacgtcatcccatctatgaaatacagtgtggaattaacgctatctttcagatcagcaggtccaaaggtagtattggaagtgtcttcttcacgcagaactgctttcaaaagcacaacatgcatctctgccatgagtgtgcactgctcttggctcaccagagctgcacaaaagtcctcaaagcgaaaaggagataatctcaaaacagtgccaaagttccgcagtacctcgtaaatggcaatgacattcattatatgctcattaggcaccattaaatcctcagaggacttgggaaattcaaggggcgggatgtctttttcttccaatataggagaacgaggccgatgtactcttggttttcgcctacctggagtgctgctgtaggtactatggctcctgaagctgctttccgtgcagtaactggcgtcgtcgtcgtcgtcttccatctcctccggataatcggagtcatcgtcgtcctcttccatctcatcctcctcgtcgtcctcagaatcctgggtctcctcggcgtcgccgtcctcctcctcctcctcctcggagaccatgtcctcctcttcctcctcctcctcgctctcgtggtcatcgtacaccactttgttgacggccctccgggccgcggtggtccgggccaggtggccgccgccgcccccgccccccgtcctgccgcccccgcctcctcgccccccccggcccggggcgctggtgctggggggggccggcggcggcggcggcggcttcctccggctactgctgccccccctgggcgagctcagccgcgtcttgggcgccacctcagcctgggcggcggcccacctgccccggctgctgccgcggtgccgcgagcggagccccccgatgggtccggacgtgggcggcggcggcggtggcggcggggccggggcgcagcgctccgcagcgggagccgcgggctgcttgggcggcctgccccgccggcccctcatgtcggagccgaggcggggggagaaggaaagcgaagggggaggggcgggcgcagggggggcggtggggagcgccggggccgggtggggaggcccgcggggccgggcgggaggggcccggccgacggaagcgggtggagggagaaggctcaatccgaattgctggggccccactccggatcgccttcagccgccatcttgtttcttccct

SEQ ID NO: 9370 - RNA, 8608 nt, Homo sapiens
  source 1..8608: mol_type = other RNA
aggaagccctggaggggctggaggagctggtgtcactggggggcagggtgcagctactgctgtggcctgagccaactgcatcaggtctttttctttcttaattttcaggtctctcttcagctcttcctgcacttcaatttgcagatccttgtccaggagtgctctcttcttcaggatctcggctctgagctgctctttgtgcttgaagagcagagctgacagcttagtggcattctgcttgctacgtttctgctccacactctcttcacgcttccgtttttttgctgcctgtttttcttctttatctatcttatccaaaatatacttcatcacctggttacagacaatcattctttgattctcttctctttcagctggagtcatgctctttttctgttttaaatgttctattacagcattatgcttcatcaccacctgtttctgaatgatttcactttgattagaagcttggagggtgtgttcacgcttaatttctatctgttgctgtttcttcttttgctgctgatccctgagttgctgaaccctttgcaactgctcttgcacactggctgcctgcactgtaaccacattctgaatctggtgagtctgcacagcactgctttgctgaatttggataggtaactggagtttgatttgctggggcacaccactttgctgagcctgtatctgagccacaacctgtgactggatctgagagagaacctggacttgttgttgcagctgaggcacagcaatgacttggggctgtggctgctgtatttgtagctgaggacgggatggggatgaaacagtaacttgatttaaagtttgtcctgatgaaagagtttgagttgaagactgtacctggggttgtgactgtggctggccttgggaaggtatctgaagagatgtatgtggttgaattggaatcggttgtgaggttgtagtctgaacctgggattgttgtccaggagacagttgggatggagttgatggacgtattcgagtctgtgatggactttggacacgaacaggagactgtccttggacattactttgaggctgagactgtgctgcaacttggggcttggatgactgtgcgtgggtgggttgtgcttcagaagggacatgggatgaaacagttgtttgggtctgaacttcaggctgagtctgaacttcaggctgagctggggactggggctgggtttggggctggggctgagctgaaggctgagcagtctgtggctgggcttctgctggacccacacttgatgactgagctggtggcagggttttgtcttgatgtacctgcatctggggtgacagtttactctgcctttgttcacctgtacctgctgctgtcgtggaaacagtggtggtggtggtgctggctgtggtggctgttgttgccaatggggtaaagaggaatcgctgaacagtaccatttggcattgcagcttgcattagctgctggcctgggcctgggagtacagtcaccccttgaggtatcaactgcaactgtccagtagtttgaccttgtccttgaattactactgtcaaaccttgattgccaccgtggccctgtgttaactgagtaagttgagccatggtgagcttcacttgtccttgttgggggcgagggggttgtgaggctgaagactgtatatttgaagtggacgttgctgaagttaagcttttctgcccaggtgttgaggaaaccgtgttaggggcggagactgcagtggagacaggctgccccctgatgatttgagtcatcacttgctgaggagcacctggctgtaccatcacaggtgttcgaataattgcctttcctagtgttgactgttggagtggtgttctaatcacggtcataccagggcgaatctgaggccctgtgattacttgtgaattgcttgtggttcctccagagcctgaggtattgggcctaattgtgactgttgctgtcctgggctggaatgaagtaaaggtttgctgactggtacctgtacttgatggaatgatacccaggactttctgctgtacttgaacaacgcctccttgtgttgctggcacatttacagcgacaatcttgctgtttgcaggaagtggcagtttggtaattacttttcctgccatagtgactggattgcctgtaatttggaacgtctgacctgtgctggcaatggttgtagcagatgtggcagctgtgctggtggctgaatttgactggccttgcttaacccatgtagcaaaggtttgatgaaagttcttgttttgttggaatgttactgtagctggagatccaactttagtagttagtaccattttggttccagttgtaactgagccacttatgggggccaccataaccttctgtgctggagagatggtgctggttgtactgcttgttggggaagtagtggaagttgcaatcactgtcggcttctgctgctccagtcgtttcttagcctgttgctcaactgcttgtgccttttctttctccactctctcagcaaatgccctgatctcccacaattccagttcttcttctgctacccaggtttcaataataacagggccagtttgcttgggcgtttctggtctctttggccgcagtgcacttgatcgaaggcctttcctctgaggtgtaggcgtttcttttggtgtttctggaactccaatgggacaaatgattttcctgatacaatattcagatcgaatgccataaggaccaacatctctcctcttaattatttctgttgttgtgatttcagtttcggatgtttctgtccgtgtagtccctcctcctggaggagccttggccgccatatcatcccatctcaaacttgcccacagtaaccgtaacatcaggctcactccagctaaggactttactgtctgaagtctatacctccaagtgatgccaaaggtcggtctaggagaaggatatggccatatatccaaagcaggttttgcattgtaattaaaataagggacctctcggattcctccttttcgggccaacttttttaagtcatcattaggcaaaacaaaaatgctcttcttgctgctcttggtaacaaattttctataggatggcagagctgtacctgaacgagtcttctttggtcttgaaaatttcatcagtttcactttgtctcgtgtggaatactctttgctcacagtcatagatgtaaccagtgtgcctcccgtggtggtcagggagtctgtcactgtcgtggtgaccacggttttgctctgctcctttacagagatgatgtccacactgccgcctgtggagggtgtggaaagcttggtcactgttgtagtggtggttgtgacagtggattttgcacaattttctgtggaagaaaccacagtttgcttatcgcctttttctaccttgatcacagtttttgattctgtggccactgtggaggtcatcgtggtgacttctgtgatgacggtttttcttttagattctccattgacattttcatttttgttgatgggcagaccattttcatcaataaagtcattactgagattagattcctcttcagaagtaataggtgatgaagtaactttcttaacttctgaggtttctatttccatatcttctacctgattaactgaattgctttctggacaagatgctgagggtgtggtcgtctgtgtactgtcagactctttggttgatggcagggtctcaaggctatctcggtagttaccttcagcatctgaagaactcagcaaatgcgattttgtttcggagctgtttctttcattaaaatcttccatgatgacatcaccattaatgaatggccttatagcagattctttaacagtcaatgatttaatatcattctcagggattattttatttatattattaacctttggttcaacattaccacttactactctactctcagaaatttctttcaagcattcacctttcaaatatattttgggtttattatcttttccatttatttgaaatgtacttgttctctgtcctttcttttcagactctcgattttcattattctttttgtcagtggtattttttagctttatttgatcactacatttattaactggtctctcctctaatttcttctgctgacttggttttttaccatttgcttcagtccccttgaccggcagcctgtcctcacagtttccagtggactcaccagaaaccaactcacactttaacggctccaagacttcaacatcttgttctcgagttctgaactgttcagaaatgctttcattgctattctgaacaatcatatcttcttcactgctatcctgaatagacacggtatcagaactattttccaaagtgctattagattcagagtcacatcccagttttccttcaaagtccattgctcttgacagaggtgtggcatctctgtcattggtacttttaggcactgatgaatgtaaagcactcttggaagaagaaacaatggtgtcactttcctcctgtatgagcggttttttgttcttacagatcaaagtaccaatatcatctgcactggctagtttagagtcatcgatgaaaaaatcatttccttttgttttactcttactgggttcctggcctctactggcaaggtcagagactttttcttctatgtcattttcaatggaattttgtttcggacattttgtttctgggctccgaatggagacatcatctaacactcgatcttttggataaagtttgtttgtggtatgactaggatcactcattctaagaactgaggaatcactttctgaacatccctgaatcaagtcctcaggttgatcattatttgcatttgggctctgttcttgtctcatcgagtcactctgacacccttcttttgctttcgttattactggtgattcagagagattttttgaagaatttgtagaagtctttcctatacccttaattccaccctccaacttgattttttcgagtcgctgtttttcttccagtgtaaactgtttaattctcctttcaagaagtccatctagtttggatgattttgttttctttttgtaactagtccttagatgaaaaccctcactaacattgaccacatctacttgagaactctcctgacaatttacatgtgactctgttttcatgtcatcgtctacttccattggttcttccttgcagggtttatcactgtcagaatctaagagctccttcacatcttggtccttcttctcagtaatctttgagatatccatttcattttggtctgctccttttgcagcatctgaaccttttacctcatctttttcagaatcaggctctatttttattttttttggacttcgtgaacattttcttttatctgactcatccatattttcatccatattatttttggttccttctaacgactttctgtaattcacattagtattgcctggcaatttaggaacaaacctataaacatgagttttactaatccagctccaaccaccatatcctgtcactctgtactcttcacctttttgtttccaaacctgatgcttaactggaaatgtgtattttacccatgtcgcttgctgcatcgtttcttcttcttcctgtttcttctctttttttttgactttctccttttcttctctttcaattgatgtcatccggtgtaacctggtatgtcctaaagattctcgccatattggtagcatcacaactggtttaactgcacactccaaaatggctaaagccaatgcaaattctctgggtttgctacacatctgaactgccttgatccaatttgccctatgtgatgcccagttgggatgaagaaaggatgaagggatgttgttttctaattgggtgatagtcagtctcagagtagatatggtaagaactttggacccatggacagaaccgttccatttgaactctcctgctggagtcagacagaacttatgtgcaagatgccttctcttatcatggtcttctctgtgctggtgcttattcaaagcaaatgaattggtggagtattgattgtggtagacgcgatacttcccttcttgacccaatttaaaataattgttgatatttcctttcatgatcacttcctttttggtgctcaaccgtgaaatttctccttgagagttaactaccagtacctctttgccctccttaaataatttatttgcttcatgtgcagcggctgccacctgctggctcttcagctgactaagtttgctatctggattccgcaatctggtgatgattcgagttgagccagatgctccttttccagctccaggagattcacttagctccccgttggacttctccgatttgaaatcacctggcacatcctgggggagctcagatgccaccttcttctctgccatgttgctgctatcgggggtttctgagagacaccccacagggctcctcccttcagagggactagtctcttctgaagttgcatttgttgtgttgtcgccaagatttgctgacacagagttacctttatccccaacttctgttggctcctcagattttccttgctcagggtcatcatctggtgttttgtcgtcactgtctttttcaagggactggtcttcaaattcttctctgtttttctcagcatctttagagtcattctcagtctcattcttgtctttttctgtttcttctgggcttttaacattatcaatgtctccctttttggctcttatggattccaaaatttcttcattagctgccgccagaaaggatttgttactgccccgagccttattggtcaggtcttcagttatgtccatgtgtcggtggatttcttcacgcatttcttctagaattttgcagagttctgcttcccaataatctttgtctagacagtcaattaattctgcaagttggacctttgtgctgtaataccaaattttcttttcattttcattttctgtatcttcttctattatgagtcttcggttcaagaaccagtatttcctccgacttctatcatatccaataggttcatgtcgaatatatggtttatttttttggatttcagcaacacagtcagtcacaccaggcaccttgtgtgctacacagacttcacactgccactcgtcctctggcacctcctcaagaggtggcttcacacattccaaatggtatactgctgaacatgtctcacagcaaagcaaatccccaagtttgtgacaaaccctacaatggtcatcatactgtatcaccccttcagacatcaattcctctcgagcaatatttgttgtaagaaactgatcgactagaaactgtagaactttgatcttgttctctactggtccatatgggtagtcctctgcctcttggtaaggaagaacgtgatggtactccttatcactctcacagtacacccgcagcacctctggccacgtcatcccatctatgaaatacagtgtggaattaacgctatctttcagatcagcaggtccaaaggtagtattggaagtgtcttcttcacgcagaactgctttcaaaagcacaacatgcatctctgccatgagtgtgcactgctcttggctcaccagagctgcacaaaagtcctcaaagcgaaaaggagataatctcaaaacagtgccaaagttccgcagtacctcgtaaatggcaatgacattcattatatgctcattaggcaccattaaatcctcagaggacttgggaaattcaaggggcgggatgtctttttcttccaatataggagaacgaggccgatgtactcttggttttcgcctacctggagtgctgctgtaggtactatggctcctgaagctgctttccgtgcagtaactggcgtcgtcgtcgtcgtcttccatctcctccggataatcggagtcatcgtcgtcctcttccatctcatcctcctcgtcgtcctcagaatcctgggtctcctcggcgtcgccgtcctcctcctcctcctcctcggagaccatgtcctcctcttcctcctcctcctcgctctcgtggtcatcgtacaccactttgttgacggccctccgggccgcggtggtccgggccaggtggccgccgccgcccccgccccccgtcctgccgcccccgcctcctcgccccccccggcccggggcgctggtgctggggggggccggcggcggcggcggcggcttcctccggctactgctgccccccctgggcgagctcagccgcgtcttgggcgccacctcagcctgggcggcggcccacctgccccggctgctgccgcggtgccgcgagcggagccccccgatgggtccggacgtgggcggcggcggcggtggcggcggggccggggcgcagcgctccgcagcgggagccgcgggctgcttgggcggcctgccccgccggcccctcatgtcggagccgaggcggggggagaaggaaagcgaagggggaggggcgggcgcagggggggcggtggggagcgccggggccgggtggggaggcccgcggggccgggcgggaggggcccggccgacggaagcgggtggagggagaaggctcaatccgaattgctggggccccactccggatcgccttcagccgccatcttgtttcttccct

SEQ ID NO: 9371 - RNA, 5926 nt, Homo sapiens
  source 1..5926: mol_type = other RNA
aggaagccctggaggggctggaggagctggtgtcactggggggcagggtgcagctactgctgtggcctgagccaactgcatcaggtctttttctttcttaattttcaggtctctcttcagctcttcctgcacttcaatttgcagatccttgtccaggagtgctctcttcttcaggatctcggctctgagctgctctttgtgcttgaagagcagagctgacagcttagtggcattctgcttgctacgtttctgctccacactctcttcacgcttccgtttttttgctgcctgtttttcttctttatctatcttatccaaaatatacttcatcacctggttacagacaatcattctttgattctcttctctttcagctggagtcatgctctttttctgttttaaatgttctattacagcattatgcttcatcaccacctgtttctgaatgatttcactttgattagaagcttggagggtgtgttcacgcttaatttctatctgttgctgtttcttcttttgctgctgatccctgagttgctgaaccctttgcaactgctcttgcacactggctgcctgcactgtaaccacattctgaatctggtgagtctgcacagcactgctttgctgaatttggataggtaactggagtttgatttgctggggcacaccactttgctgagcctgtatctgagccacaacctgtgactggatctgagagagaacctggacttgttgttgcagctgaggcacagcaatgacttggggctgtggctgctgtatttgtagctgaggacgggatggggatgaaacagtaacttgatttaaagtttgtcctgatgaaagagtttgagttgaagactgtacctggggttgtgactgtggctggccttgggaaggtatctgaagagatgtatgtggttgaattggaatcggttgtgaggttgtagtctgaacctgggattgttgtccaggagacagttgggatggagttgatggacgtattcgagtctgtgatggactttggacacgaacaggagactgtccttggacattactttgaggctgagactgtgctgcaacttggggcttggatgactgtgcgtgggtgggttgtgcttcagaagggacatgggatgaaacagttgtttgggtctgaacttcaggctgagtctgaacttcaggctgagctggggactggggctgggtttggggctggggctgagctgaaggctgagcagtctgtggctgggcttctgctggacccacacttgatgactgagctggtggcagggttttgtcttgatgtacctgcatctggggtgacagtttactctgcctttgttcacctgtacctgctgctgtcgtggaaacagtggtggtggtggtgctggctgtggtggctgttgttgccaatggggtaaagaggaatcgctgaacagtaccatttggcattgcagcttgcattagctgctggcctgggcctgggagtacagtcaccccttgaggtatcaactgcaactgtccagtagtttgaccttgtccttgaattactactgtcaaaccttgattgccaccgtggccctgtgttaactgagtaagttgagccatggtgagcttcacttgtccttgttgggggcgagggggttgtgaggctgaagactgtatatttgaagtggacgttgctgaagttaagcttttctgcccaggtgttgaggaaaccgtgttaggggcggagactgcagtggagacaggctgccccctgatgatttgagtcatcacttgctgaggagcacctggctgtaccatcacaggtgttcgaataattgcctttcctagtgttgactgttggagtggtgttctaatcacggtcataccagggcgaatctgaggccctgtgattacttgtgaattgcttgtggttcctccagagcctgaggtattgggcctaattgtgactgttgctgtcctgggctggaatgaagtaaaggtttgctgactggtacctgtacttgatggaatgatacccaggactttctgctgtacttgaacaacgcctccttgtgttgctggcacatttacagcgacaatcttgctgtttgcaggaagtggcagtttggtaattacttttcctgccatagtgactggattgcctgtaatttggaacgtctgacctgtgctggcaatggttgtagcagatgtggcagctgtgctggtggctgaatttgactggccttgcttaacccatgtagcaaaggtttgatgaaagttcttgttttgttggaatgttactgtagctggagatccaactttagtagttagtaccattttggttccagttgtaactgagccacttatgggggccaccataaccttctgtgctggagagatggtgctggttgtactgcttgttggggaagtagtggaagttgcaatcactgtcggcttctgctgctccagtcgtttcttagcctgttgctcaactgcttgtgccttttctttctccactctctcagcaaatgccctgatctcccacaattccagttcttcttctgctacccaggtttcaataataacagggccagtttgcttgggcgtttctggtctctttggccgcagtgcacttgatcgaaggcctttcctctgaggtgtaggcgtttcttttggtgtttctggaactccaatgggacaaatgattttcctgatacaatattcagatcgaatgccataaggaccaacatctctcctcttaattatttctgttgttgtgatttcagtttcggatgtttctgtccgtgtagtccctcctcctggaggagccttggccgccatatcatcccatctcaaacttgcccacagtaaccgtaacatcaggctcactccagctaaggactttactgtctgaagtctatacctccaagtgatgccaaaggtcggtctaggagaaggatatggccatatatccaaagcaggttttgcattgtaattaaaataagggacctctcggattcctccttttcgggccaacttttttaagtcatcattaggcaaaacaaaaatgctcttcttgctgctcttggtaacaaattttctataggatggcagagctgtacctgaacgagtcttctttggtcttgaaaatttcatcagtttcactttgtctcgtgtggaatactctttgctcacagtcatagatgtaaccagtgtgcctcccgtggtggtcagggagtctgtcactgtcgtggtgaccacggttttgctctgctcctttacagagatgatgtccacactgccgcctgtggagggtgtggaaagcttggtcactgttgtagtggtggttgtgacagtggattttgcacaattttctgtggaagaaaccacagtttgcttatcgcctttttctaccttgatcacagtttttgattctgtggccactgtggaggtcatcgtggtgacttctgtgatgacggtttttcttttagattctccattgacattttcatttttgttgatgggcagaccattttcatcaataaagtcattactgagattagattcctcttcagaagtaataggtgatgaagtaactttcttaacttctgaggtttctatttccatatcttctacctgattaactgaattgctttctggacaagatgctgagggtgtggtcgtctgtgtactgtcagactctttggttgatggcagggtctcaaggctatctcggtagttaccttcagcatctgaagaactcagcaaatgcgattttgtttcggagctgtttctttcattaaaatcttccatgatgacatcaccattaatgaatggccttatagcagattctttaacagtcaatgatttaatatcattctcagggattattttatttatattattaacctttggttcaacattaccacttactactctactctcagaaatttctttcaagcattcacctttcaaatatattttgggtttattatcttttccatttatttgaaatgtacttgttctctgtcctttcttttcagactctcgattttcattattctttttgtcagtggtattttttagctttatttgatcactacatttattaactggtctctcctctaatttcttctgctgacttggttttttaccatttgcttcagtccccttgaccggcagcctgtcctcacagtttccagtggactcaccagaaaccaactcacactttaacggctccaagacttcaacatcttgttctcgagttctgaactgttcagaaatgctttcattgctattctgaacaatcatatcttcttcactgctatcctgaatagacacggtatcagaactattttccaaagtgctattagattcagagtcacatcccagttttccttcaaagtccattgctcttgacagaggtgtggcatctctgtcattggtacttttaggcactgatgaatgtaaagcactcttggaagaagaaacaatggtgtcactttcctcctgtatgagcggttttttgttcttacagatcaaagtaccaatatcatctgcactggctagtttagagtcatcgatgaaaaaatcatttccttttgttttactcttactgggttcctggcctctactggcaaggtcagagactttttcttctatgtcattttcaatggaattttgtttcggacattttgtttctgggctccgaatggagacatcatctaacactcgatcttttggataaagtttgtttgtggtatgactaggatcactcattctaagaactgaggaatcactttctgaacatccctgaatcaagtcctcaggttgatcattatttgcatttgggctctgttcttgtctcatcgagtcactctgacacccttcttttgctttcgttattactggtgattcagagagattttttgaagaatttgtagaagtctttcctatacccttaattccaccctccaacttgattttttcgagtcgctgtttttcttccagtgtaaactgtttaattctcctttcaagaagtccatctagtttggatgattttgttttctttttgtaactagtccttagatgaaaaccctcactaacattgaccacatctacttgagaactctcctgacaatttacatgtgactctgttttcatgtcatcgtctacttccattggttcttccttgcagggtttatcactgtcagaatctaagagctccttcacatcttggtccttcttctcagtaatctttgagatatccatttcattttggtctgctccttttgcagcatctgaaccttttacctcatctttttcagaatcaggctctatttttattttttttggacttcgtgaacattttcttttatctgactcatccatattttcatccatattatttttggttccttctaacgactttctgtaattcacattagtattgcctggcaatttaggaacaaacctataaacatgagttttactaatccagctccaaccaccatatcctgtcactctgtactcttcacctttttgtttccaaacctgatgcttaactggaaatgtgtattttacccatgtcgcttgctgcatcgtttcttcttcttcctgtttcttctctttttttttgactttctccttttcttctctttcaattgatgtcatccggtgtaaccttcttggcatctaatgagatgatcaaaaggtttcctttcttcaacttttttctttttaagacagcatcttgctctgttgctcaggatggagtgcactggtgcgatctcagctcattgcaacctctgcctcccaggttcaagtggttctcctgcctcagcctcctagtagctgggactaaaggcatgcaacaccatgcctggctaatttttagtagagatggggtttcaccacattggccatgctggtcttaaac

SEQ ID NO: 9372 - RNA, 8257 nt, Homo sapiens
  source 1..8257: mol_type = other RNA
aggaagccctggaggggctggaggagctggtgtcactggggggcagggtgcagctactgctgtggcctgagccaactgcatcaggtctttttctttcttaattttcaggtctctcttcagctcttcctgcacttcaatttgcagatccttgtccaggagtgctctcttcttcaggatctcggctctgagctgctctttgtgcttgaagagcagagctgacagcttagtggcattctgcttgctacgtttctgctccacactctcttcacgcttccgtttttttgctgcctgtttttcttctttatctatcttatccaaaatatacttcatcacctggttacagacaatcattctttgattctcttctctttcagctggagtcatgctctttttctgttttaaatgttctattacagcattatgcttcatcaccacctgtttctgaatgatttcactttgattagaagcttggagggtgtgttcacgcttaatttctatctgttgctgtttcttcttttgctgctgatccctgagttgctgaaccctttgcaactgctcttgcacactggctgcctgcactgtaaccacattctgaatctggtgagtctgcacagcactgctttgctgaatttggataggtaactggagtttgatttgctggggcacaccactttgctgagcctgtatctgagccacaacctgtgactggatctgagagagaacctggacttgttgttgcagctgaggcacagcaatgacttggggctgtggctgctgtatttgtagctgaggacgggatggggatgaaacagtaacttgatttaaagtttgtcctgatgaaagagtttgagttgaagactgtacctggggttgtgactgtggctggccttgggaaggtatctgaagagatgtatgtggttgaattggaatcggttgtgaggttgtagtctgaacctgggattgttgtccaggagacagttgggatggagttgatggacgtattcgagtctgtgatggactttggacacgaacaggagactgtccttggacattactttgaggctgagactgtgctgcaacttggggcttggatgactgtgcgtgggtgggttgtgcttcagaagggacatgggatgaaacagttgtttgggtctgaacttcaggctgagtctgaacttcaggctgagctggggactggggctgggtttggggctggggctgagctgaaggctgagcagtctgtggctgggcttctgctggacccacacttgatgactgagctggtggcagggttttgtcttgatgtacctgcatctggggtgacagtttactctgcctttgttcacctgtacctgctgctgtcgtggaaacagtggtggtggtggtgctggctgtggtggctgttgttgccaatggggtaaagaggaatcgctgaacagtaccatttggcattgcagcttgcattagctgctggcctgggcctgggagtacagtcaccccttgaggtatcaactgcaactgtccagtagtttgaccttgtccttgaattactactgtcaaaccttgattgccaccgtggccctgtgttaactgagtaagttgagccatggtgagcttcacttgtccttgttgggggcgagggggttgtgaggctgaagactgtatatttgaagtggacgttgctgaagttaagcttttctgcccaggtgttgaggaaaccgtgttaggggcggagactgcagtggagacaggctgccccctgatgatttgagtcatcacttgctgaggagcacctggctgtaccatcacaggtgttcgaataattgcctttcctagtgttgactgttggagtggtgttctaatcacggtcataccagggcgaatctgaggccctgtgattacttgtgaattgcttgtggttcctccagagcctgaggtattgggcctaattgtgactgttgctgtcctgggctggaatgaagtaaaggtttgctgactggtacctgtacttgatggaatgatacccaggactttctgctgtacttgaacaacgcctgaatttgactggccttgcttaacccatgtagcaaaggtttgatgaaagttcttgttttgttggaatgttactgtagctggagatccaactttagtagttagtaccattttggttccagttgtaactgagccacttatgggggccaccataaccttctgtgctggagagatggtgctggttgtactgcttgttggggaagtagtggaagttgcaatcactgtcggcttctgctgctccagtcgtttcttagcctgttgctcaactgcttgtgccttttctttctccactctctcagcaaatgccctgatctcccacaattccagttcttcttctgctacccaggtttcaataataacagggccagtttgcttgggcgtttctggtctctttggccgcagtgcacttgatcgaaggcctttcctctgaggtgtaggcgtttcttttggtgtttctggaactccaatgggacaaatgattttcctgatacaatattcagatcgaatgccataaggaccaacatctctcctcttaattatttctgttgttgtgatttcagtttcggatgtttctgtccgtgtagtccctcctcctggaggagccttggccgccatatcatcccatctcaaacttgcccacagtaaccgtaacatcaggctcactccagctaaggactttactgtctgaagtctatacctccaagtgatgccaaaggtcggtctaggagaaggatatggccatatatccaaagcaggttttgcattgtaattaaaataagggacctctcggattcctccttttcgggccaacttttttaagtcatcattaggcaaaacaaaaatgctcttcttgctgctcttggtaacaaattttctataggatggcagagctgtacctgaacgagtcttctttggtcttgaaaatttcatcagtttcactttgtctcgtgtggaatactctttgctcacagtcatagatgtaaccagtgtgcctcccgtggtggtcagggagtctgtcactgtcgtggtgaccacggttttgctctgctcctttacagagatgatgtccacactgccgcctgtggagggtgtggaaagcttggtcactgttgtagtggtggttgtgacagtggattttgcacaattttctgtggaagaaaccacagtttgcttatcgcctttttctaccttgatcacagtttttgattctgtggccactgtggaggtcatcgtggtgacttctgtgatgacggtttttcttttagattctccattgacattttcatttttgttgatgggcagaccattttcatcaataaagtcattactgagattagattcctcttcagaagtaataggtgatgaagtaactttcttaacttctgaggtttctatttccatatcttctacctgattaactgaattgctttctggacaagatgctgagggtgtggtcgtctgtgtactgtcagactctttggttgatggcagggtctcaaggctatctcggtagttaccttcagcatctgaagaactcagcaaatgcgattttgtttcggagctgtttctttcattaaaatcttccatgatgacatcaccattaatgaatggccttatagcagattctttaacagtcaatgatttaatatcattctcagggattattttatttatattattaacctttggttcaacattaccacttactactctactctcagaaatttctttcaagcattcacctttcaaatatattttgggtttattatcttttccatttatttgaaatgtacttgttctctgtcctttcttttcagactctcgattttcattattctttttgtcagtggtattttttagctttatttgatcactacatttattaactggtctctcctctaatttcttctgctgacttggttttttaccatttgcttcagtccccttgaccggcagcctgtcctcacagtttccagtggactcaccagaaaccaactcacactttaacggctccaagacttcaacatcttgttctcgagttctgaactgttcagaaatgctttcattgctattctgaacaatcatatcttcttcactgctatcctgaatagacacggtatcagaactattttccaaagtgctattagattcagagtcacatcccagttttccttcaaagtccattgctcttgacagaggtgtggcatctctgtcattggtacttttaggcactgatgaatgtaaagcactcttggaagaagaaacaatggtgtcactttcctcctgtatgagcggttttttgttcttacagatcaaagtaccaatatcatctgcactggctagtttagagtcatcgatgaaaaaatcatttccttttgttttactcttactgggttcctggcctctactggcaaggtcagagactttttcttctatgtcattttcaatggaattttgtttcggacattttgtttctgggctccgaatggagacatcatctaacactcgatcttttggataaagtttgtttgtggtatgactaggatcactcattctaagaactgaggaatcactttctgaacatccctgaatcaagtcctcaggttgatcattatttgcatttgggctctgttcttgtctcatcgagtcactctgacacccttcttttgctttcgttattactggtgattcagagagattttttgaagaatttgtagaagtctttcctatacccttaattccaccctccaacttgattttttcgagtcgctgtttttcttccagtgtaaactgtttaattctcctttcaagaagtccatctagtttggatgattttgttttctttttgtaactagtccttagatgaaaaccctcactaacattgaccacatctacttgagaactctcctgacaatttacatgtgactctgttttcatgtcatcgtctacttccattggttcttccttgcagggtttatcactgtcagaatctaagagctccttcacatcttggtccttcttctcagtaatctttgagatatccatttcattttggtctgctccttttgcagcatctgaaccttttacctcatctttttcagaatcaggctctatttttattttttttggacttcgtgaacattttcttttatctgactcatccatattttcatccatattatttttggttccttctaacgactttctgtaattcacattagtattgcctggcaatttaggaacaaacctataaacatgagttttactaatccagctccaaccaccatatcctgtcactctgtactcttcacctttttgtttccaaacctgatgcttaactggaaatgtgtattttacccatgtcgcttgctgcatcgtttcttcttcttcctgtttcttctctttttttttgactttctccttttcttctctttcaattgatgtcatccggtgtaacctggtatgtcctaaagattctcgccatattggtagcatcacaactggtttaactgcacactccaaaatggctaaagccaatgcaaattctctgggtttgctacacatctgaactgccttgatccaatttgccctatgtgatgcccagttgggatgaagaaaggatgaagggatgttgttttctaattgggtgatagtcagtctcagagtagatatggtaagaactttggacccatggacagaaccgttccatttgaactctcctgctggagtcagacagaacttatgtgcaagatgccttctcttatcatggtcttctctgtgctggtgcttattcaaagcaaatgaattggtggagtattgattgtggtagacgcgatacttcccttcttgacccaatttaaaataattgttgatatttcctttcatgatcacttcctttttggtgctcaaccgtgaaatttctccttgagagttaactaccagtacctctttgccctccttaaataatttatttgcttcatgtgcagcggctgccacctgctggctcttcagctgactaagtttgctatctggattccgcaatctggtgatgattcgagttgagccagatgctccttttccagctccaggagattcacttagctccccgttggacttctccgatttgaaatcaccctcagattttccttgctcagggtcatcatctggtgttttgtcgtcactgtctttttcaagggactggtcttcaaattcttctctgtttttctcagcatctttagagtcattctcagtctcattcttgtctttttctgtttcttctgggcttttaacattatcaatgtctccctttttggctcttatggattccaaaatttcttcattagctgccgccagaaaggatttgttactgccccgagccttattggtcaggtcttcagttatgtccatgtgtcggtggatttcttcacgcatttcttctagaattttgcagagttctgcttcccaataatctttgtctagacagtcaattaattctgcaagttggacctttgtgctgtaataccaaattttcttttcattttcattttctgtatcttcttctattatgagtcttcggttcaagaaccagtatttcctccgacttctatcatatccaataggttcatgtcgaatatatggtttatttttttggatttcagcaacacagtcagtcacaccaggcaccttgtgtgctacacagacttcacactgccactcgtcctctggcacctcctcaagaggtggcttcacacattccaaatggtatactgctgaacatgtctcacagcaaagcaaatccccaagtttgtgacaaaccctacaatggtcatcatactgtatcaccccttcagacatcaattcctctcgagcaatatttgttgtaagaaactgatcgactagaaactgtagaactttgatcttgttctctactggtccatatgggtagtcctctgcctcttggtaaggaagaacgtgatggtactccttatcactctcacagtacacccgcagcacctctggccacgtcatcccatctatgaaatacagtgtggaattaacgctatctttcagatcagcaggtccaaaggtagtattggaagtgtcttcttcacgcagaactgctttcaaaagcacaacatgcatctctgccatgagtgtgcactgctcttggctcaccagagctgcacaaaagtcctcaaagcgaaaaggagataatctcaaaacagtgccaaagttccgcagtacctcgtaaatggcaatgacattcattatatgctcattaggcaccattaaatcctcagaggacttgggaaattcaaggggcgggatgtctttttcttccaatataggagaacgaggccgatgtactcttggttttcgcctacctggagtgctgctgtaggtactatggctcctgaagctgctttccgtgcagtaactggcgtcgtcgtcgtcgtcttccatctcctccggataatcggagtcatcgtcgtcctcttccatctcatcctcctcgtcgtcctcagaatcctgggtctcctcggcgtcgccgtcctcctcctcctcctcctcggagaccatgtcctcctcttcctcctcctcctcgctctcgtggtcatcgtacaccactttgttgacggccctccgggccgcggtggtccgggccaggtggccgccgccgcccccgccccccgtcctgccgcccccgcctcctcgccccccccggcccggggcgctggtgctggggggggccggcggcggcggcggcggcttcctccggctactgctgccccccctgggcgagctcagccgcgtcttgggcgccacctcagcctgggcggcggcccacctgccccggctgctgccgcggtgccgcgagcggagccccccgatgggtccggacgtgggcggcggcggcggtggcggcggggccggggcgcagcgctccgcagcgggagccgcgggctgcttgggcggcctgccccgccggcccctcatgtcggagccgaggcggggggagaaggaaagcgaagggggaggggcgggcgcagggggggcggtggggagcgccggggccgggtggggaggcccgcggggccgggcgggaggggcccggccgacggaagcgggtggagggagaaggctcaatccgaattgctggggccccactccggatcgccttcagccgccatcttgtttcttccct

SEQ ID NO: 9373 - RNA, 8274 nt, Homo sapiens
  source 1..8274: mol_type = other RNA
aggaagccctggaggggctggaggagctggtgtcactggggggcagggtgcagctactgctgtggcctgagccaactgcatcaggtctttttctttcttaattttcaggtctctcttcagctcttcctgcacttcaatttgcagatccttgtccaggagtgctctcttcttcaggatctcggctctgagctgctctttgtgcttgaagagcagagctgacagcttagtggcattctgcttgctacgtttctgctccacactctcttcacgcttccgtttttttgctgcctgtttttcttctttatctatcttatccaaaatatacttcatcacctggttacagacaatcattctttgattctcttctctttcagctggagtcatgctctttttctgttttaaatgttctattacagcattatgcttcatcaccacctgtttctgaatgatttcactttgattagaagcttggagggtgtgttcacgcttaatttctatctgttgctgtttcttcttttgctgctgatccctgagttgctgaaccctttgcaactgctcttgcacactggctgcctgcactgtaaccacattctgaatctggtgagtctgcacagcactgctttgctgaatttggataggtaactggagtttgatttgctggggcacaccactttgctgagcctgtatctgagccacaacctgtgactggatctgagagagaacctggacttgttgttgcagctgaggcacagcaatgacttggggctgtggctgctgtatttgtagctgaggacgggatggggatgaaacagtaacttgatttaaagtttgtcctgatgaaagagtttgagttgaagactgtacctggggttgtgactgtggctggccttgggaaggtatctgaagagatgtatgtggttgaattggaatcggttgtgaggttgtagtctgaacctgggattgttgtccaggagacagttgggatggagttgatggacgtattcgagtctgtgatggactttggacacgaacaggagactgtccttggacattactttgaggctgagactgtgctgcaacttggggcttggatgactgtgcgtgggtgggttgtgcttcagaagggacatgggatgaaacagttgtttgggtctgaacttcaggctgagtctgaacttcaggctgagctggggactggggctgggtttggggctggggctgagctgaaggctgagcagtctgtggctgggcttctgctggacccacacttgatgactgagctggtggcagggttttgtcttgatgtacctgcatctggggtgacagtttactctgcctttgttcacctgtacctgctgctgtcgtggaaacagtggtggtggtggtgctggctgtggtggctgttgttgccaatggggtaaagaggaatcgctgaacagtaccatttggcattgcagcttgcattagctgctggcctgggcctgggagtacagtcaccccttgaggtatcaactgcaactgtccagtagtttgaccttgtccttgaattactactgtcaaaccttgattgccaccgtggccctgtgttaactgagtaagttgagccatggtgagcttcacttgtccttgttgggggcgagggggttgtgaggctgaagactgtatatttgaagtggacgttgctgaagttaagcttttctgcccaggtgttgaggaaaccgtgttaggggcggagactgcagtggagacaggctgccccctgatgatttgagtcatcacttgctgaggagcacctggctgtaccatcacaggtgttcgaataattgcctttcctagtgttgactgttggagtggtgttctaatcacggtcataccagggcgaatctgaggccctgtgattacttgtgaattgcttgtggttcctccagagcctgaggtattgggcctaattgtgactgttgctgtcctgggctggaatgaagtaaaggtttgctgactggtacctgtacttgatggaatgatacccaggactttctgctgtacttgaacaacgcctgaatttgactggccttgcttaacccatgtagcaaaggtttgatgaaagttcttgttttgttggaatgttactgtagctggagatccaactttagtagttagtaccattttggttccagttgtaactgagccacttatgggggccaccataaccttctgtgctggagagatggtgctggttgtactgcttgttggggaagtagtggaagttgcaatcactgtcggcttctgctgctccagtcgtttcttagcctgttgctcaactgcttgtgccttttctttctccactctctcagcaaatgccctgatctcccacaattccagttcttcttctgctacccaggtttcaataataacagggccagtttgcttgggcgtttctggtctctttggccgcagtgcacttgatcgaaggcctttcctctgaggtgtaggcgtttcttttggtgtttctggaactccaatgggacaaatgattttcctgatacaatattcagatcgaatgccataaggaccaacatctctcctcttaattatttctgttgttgtgatttcagtttcggatgtttctgtccgtgtagtccctcctcctggaggagccttggccgccatatcatcccatctcaaacttgcccacagtaaccgtaacatcaggctcactccagctaaggactttactgtctgaagtctatacctccaagtgatgccaaaggtcggtctaggagaaggatatggccatatatccaaagcaggttttgcattgtaattaaaataagggacctctcggattcctccttttcgggccaacttttttaagtcatcattaggcaaaacaaaaatgctcttcttgctgctcttggtaacaaattttctataggatggcagagctgtacctgaacgagtcttctttggtcttgaaaatttcatcagtttcactttgtctcgtgtggaatactctttgctcacagtcatagatgtaaccagtgtgcctcccgtggtggtcagggagtctgtcactgtcgtggtgaccacggttttgctctgctcctttacagagatgatgtccacactgccgcctgtggagggtgtggaaagcttggtcactgttgtagtggtggttgtgacagtggattttgcacaattttctgtggaagaaaccacagtttgcttatcgcctttttctaccttgatcacagtttttgattctgtggccactgtggaggtcatcgtggtgacttctgtgatgacggtttttcttttagattctccattgacattttcatttttgttgatgggcagaccattttcatcaataaagtcattactgagattagattcctcttcagaagtaataggtgatgaagtaactttcttaacttctgaggtttctatttccatatcttctacctgattaactgaattgctttctggacaagatgctgagggtgtggtcgtctgtgtactgtcagactctttggttgatggcagggtctcaaggctatctcggtagttaccttcagcatctgaagaactcagcaaatgcgattttgtttcggagctgtttctttcattaaaatcttccatgatgacatcaccattaatgaatggccttatagcagattctttaacagtcaatgatttaatatcattctcagggattattttatttatattattaacctttggttcaacattaccacttactactctactctcagaaatttctttcaagcattcacctttcaaatatattttgggtttattatcttttccatttatttgaaatgtacttgttctctgtcctttcttttcagactctcgattttcattattctttttgtcagtggtattttttagctttatttgatcactacatttattaactggtctctcctctaatttcttctgctgacttggttttttaccatttgcttcagtccccttgaccggcagcctgtcctcacagtttccagtggactcaccagaaaccaactcacactttaacggctccaagacttcaacatcttgttctcgagttctgaactgttcagaaatgctttcattgctattctgaacaatcatatcttcttcactgctatcctgaatagacacggtatcagaactattttccaaagtgctattagattcagagtcacatcccagttttccttcaaagtccattgctcttgacagaggtgtggcatctctgtcattggtacttttaggcactgatgaatgtaaagcactcttggaagaagaaacaatggtgtcactttcctcctgtatgagcggttttttgttcttacagatcaaagtaccaatatcatctgcactggctagtttagagtcatcgatgaaaaaatcatttccttttgttttactcttactgggttcctggcctctactggcaaggtcagagactttttcttctatgtcattttcaatggaattttgtttcggacattttgtttctgggctccgaatggagacatcatctaacactcgatcttttggataaagtttgtttgtggtatgactaggatcactcattctaagaactgaggaatcactttctgaacatccctgaatcaagtcctcaggttgatcattatttgcatttgggctctgttcttgtctcatcgagtcactctgacacccttcttttgctttcgttattactggtgattcagagagattttttgaagaatttgtagaagtctttcctatacccttaattccaccctccaacttgattttttcgagtcgctgtttttcttccagtgtaaactgtttaattctcctttcaagaagtccatctagtttggatgattttgttttctttttgtaactagtccttagatgaaaaccctcactaacattgaccacatctacttgagaactctcctgacaatttacatgtgactctgttttcatgtcatcgtctacttccattggttcttccttgcagggtttatcactgtcagaatctaagagctccttcacatcttggtccttcttctcagtaatctttgagatatccatttcattttggtctgctccttttgcagcatctgaaccttttacctcatctttttcagaatcaggctctatttttattttttttggacttcgtgaacattttcttttatctgactcatccatattttcatccatattatttttggttccttctaacgactttctgtaattcacattagtattgcctggcaatttaggaacaaacctataaacatgagttttactaatccagctccaaccaccatatcctgtcactctgtactcttcacctttttgtttccaaacctgatgcttaactggaaatgtgtattttacccatgtcgcttgctgcatcgtttcttcttcttcctgtttcttctctttttttttgactttctccttttcttctctttcaattgatgtcatccggtgtaacctggtatgtcctaaagattctcgccatattggtagcatcacaactggtttaactgcacactccaaaatggctaaagccaatgcaaattctctgggtttgctacacatctgaactgccttgatccaatttgccctatgtgatgcccagttgggatgaagaaaggatgaagggatgttgttttctaattgggtgatagtcagtctcagagtagatatggtaagaactttggacccatggacagaaccgttccatttgaactctcctgctggagtcagacagaacttatgtgcaagatgccttctcttatcatggtcttctctgtgctggtgcttattcaaagcaaatgaattggtggagtattgattgtggtagacgcgatacttcccttcttgacccaatttaaaataattgttgatatttcctttcatgatcacttcctttttggtgctcaaccgtgaaatttctccttgagagttaactaccagtacctctttgccctccttaaataatttatttgcttcatgtgcagcggctgccacctgctggctcttcagctgactaagtttgctatctggattccgcaatctggtgatgattcgagttgagccagatgctccttttccagctccaggagattcacttagctccccgttggacttctccgatttgaaatcacctacctcagattttccttgctcagggtcatcatctggtgttttgtcgtcactgtctttttcaagggactggtcttcaaattcttctctgtttttctcagcatctttagagtcattctcagtctcattcttgtctttttctgtttcttctgggcttttaacattatcaatgtctccctttttggctcttatggattccaaaatttcttcattagctgccgccagaaaggatttgttactgccccgagccttattggtcaggtcttcagttatgtccatgtgtcggtggatttcttcacgcatttcttctagaattttgcagagttctgcttcccaataatctttgtctagacagtcaattaattctgcaagttggacctttgtgctgtaataccaaattttcttttcattttcattttctgtatcttcttctattatgagtcttcggttcaagaaccagtatttcctccgacttctatcatatccaataggttcatgtcgaatatatggtttatttttttggatttcagcaacacagtcagtcacaccaggcaccttgtgtgctacacagacttcacactgccactcgtcctctggcacctcctcaagaggtggcttcacacattccaaatggtatactgctgaacatgtctcacagcaaagcaaatccccaagtttgtgacaaaccctacaatggtcatcatactgtatcaccccttcagacatcaattcctctcgagcaatatttgttgtaagaaactgatcgactagaaactgtagaactttgatcttgttctctactggtccatatgggtagtcctctgcctcttggtaaggaagaacgtgatggtactccttatcactctcacagtacacccgcagcacctctggccacgtcatcccatctatgaaatacagtgtggaattaacgctatctttcagatcagcaggtccaaaggtagtattggaagtgtcttcttcacgcagaactgctttcaaaagcacaacatgcatctctgccatgagtgtgcactgctcttggctcaccagagctgcacaaaagtcctcaaagcgaaaaggagataatctcaaaacagtgccaaagttccgcagtacctcgtaaatggcaatgacattcattatatgctcattaggcaccattaaatcctcagaggacttgggaaattcaaggggcgggatgtctttttcttccaatataggagaacgaggccgatgtactcttggttttcgcctacctggagtgctgctgtaggtactatggctcctgaagctgctttccgtgcagtaactggcgtcgtcgtcgtcgtcttccatctcctccggataatcggagtcatcgtcgtcctcttccatctcatcctcctcgtcgtcctcagaatcctgggtctcctcggcgtcgccgtcctcctcctcctcctcctcggagaccatgtcctcctcttcctcctcctcctcgctctcgtggtcatcgtacaccactttgttgacggccctccgggccgcggtggtccgggccaggtggccgccgccgcccccgccccccgtcctgccgcccccgcctcctcgccccccccggcccggggcgctggtgctggggggggccggcggcggcggcggcggcttcctccggctactgctgccccccctgggcgagctcagccgcgtcttgggcgccacctcagcctgggcggcggcccacctgccccggctgctgccgcggtgccgcgagcggagccccccgatgggtccggacgtgggcggcggcggcggtggcggcggggccggggcgcagcgctccgcagcgggagccgcgggctgcttgggcggcctgccccgccggcccctcatgtcggagccgaggcggggggagaaggaaagcgaagggggaggggcgggcgcagggggggcggtggggagcgccggggccgggtggggaggcccgcggggccgggcgggaggggcccggccgacggaagcgggtggagggagaaggctcaatccgaattgctggggccccactccggatcgccttcagccgccatcttgtttcttccctctcgctcggtgact

SEQ ID NO: 9374 - RNA, 8638 nt, Homo sapiens
  source 1..8638: mol_type = other RNA
aggaagccctggaggggctggaggagctggtgtcactggggggcagggtgcagctactgctgtggcctgagccaactgcatcaggtctttttctttcttaattttcaggtctctcttcagctcttcctgcacttcaatttgcagatccttgtccaggagtgctctcttcttcaggatctcggctctgagctgctctttgtgcttgaagagcagagctgacagcttagtggcattctgcttgctacgtttctgctccacactctcttcacgcttccgtttttttgctgcctgtttttcttctttatctatcttatccaaaatatacttcatcacctggttacagacaatcattctttgattctcttctctttcagctggagtcatgctctttttctgttttaaatgttctattacagcattatgcttcatcaccacctgtttctgaatgatttcactttgattagaagcttggagggtgtgttcacgcttaatttctatctgttgctgtttcttcttttgctgctgatccctgagttgctgaaccctttgcaactgctcttgcacactggctgcctgcactgtaaccacattctgaatctggtgagtctgcacagcactgctttgctgaatttggataggtaactggagtttgatttgctggggcacaccactttgctgagcctgtatctgagccacaacctgtgactggatctgagagagaacctggacttgttgttgcagctgaggcacagcaatgacttggggctgtggctgctgtatttgtagctgaggacgggatggggatgaaacagtaacttgatttaaagtttgtcctgatgaaagagtttgagttgaagactgtacctggggttgtgactgtggctggccttgggaaggtatctgaagagatgtatgtggttgaattggaatcggttgtgaggttgtagtctgaacctgggattgttgtccaggagacagttgggatggagttgatggacgtattcgagtctgtgatggactttggacacgaacaggagactgtccttggacattactttgaggctgagactgtgctgcaacttggggcttggatgactgtgcgtgggtgggttgtgcttcagaagggacatgggatgaaacagttgtttgggtctgaacttcaggctgagtctgaacttcaggctgagctggggactggggctgggtttggggctggggctgagctgaaggctgagcagtctgtggctgggcttctgctggacccacacttgatgactgagctggtggcagggttttgtcttgatgtacctgcatctggggtgacagtttactctgcctttgttcacctgtacctgctgctgtcgtggaaacagtggtggtggtggtgctggctgtggtggctgttgttgccaatggggtaaagaggaatcgctgaacagtaccatttggcattgcagcttgcattagctgctggcctgggcctgggagtacagtcaccccttgaggtatcaactgcaactgtccagtagtttgaccttgtccttgaattactactgtcaaaccttgattgccaccgtggccctgtgttaactgagtaagttgagccatggtgagcttcacttgtccttgttgggggcgagggggttgtgaggctgaagactgtatatttgaagtggacgttgctgaagttaagcttttctgcccaggtgttgaggaaaccgtgttaggggcggagactgcagtggagacaggctgccccctgatgatttgagtcatcacttgctgaggagcacctggctgtaccatcacaggtgttcgaataattgcctttcctagtgttgactgttggagtggtgttctaatcacggtcataccagggcgaatctgaggccctgtgattacttgtgaattgcttgtggttcctccagagcctgaggtattgggcctaattgtgactgttgctgtcctgggctggaatgaagtaaaggtttgctgactggtacctgtacttgatggaatgatacccaggactttctgctgtacttgaacaacgcctgaatttgactggccttgcttaacccatgtagcaaaggtttgatgaaagttcttgttttgttggaatgttactgtagctggagatccaactttagtagttagtaccattttggttccagttgtaactgagccacttatgggggccaccataaccttctgtgctggagagatggtgctggttgtactgcttgttggggaagtagtggaagttgcaatcactgtcggcttctgctgctccagtcgtttcttagcctgttgctcaactgcttgtgccttttctttctccactctctcagcaaatgccctgatctcccacaattccagttcttcttctgctacccaggtttcaataataacagggccagtttgcttgggcgtttctggtctctttggccgcagtgcacttgatcgaaggcctttcctctgaggtgtaggcgtttcttttggtgtttctggaactccaatgggacaaatgattttcctgatacaatattcagatcgaatgccataaggaccaacatctctcctcttaattatttctgttgttgtgatttcagtttcggatgtttctgtccgtgtagtccctcctcctggaggagccttggccgccatatcatcccatctcaaacttgcccacagtaaccgtaacatcaggctcactccagctaaggactttactgtctgaagtctatacctccaagtgatgccaaaggtcggtctaggagaaggatatggccatatatccaaagcaggttttgcattgtaattaaaataagggacctctcggattcctccttttcgggccaacttttttaagtcatcattaggcaaaacaaaaatgctcttcttgctgctcttggtaacaaattttctataggatggcagagctgtacctgaacgagtcttctttggtcttgaaaatttcatcagtttcactttgtctcgtgtggaatactctttgctcacagtcatagatgtaaccagtgtgcctcccgtggtggtcagggagtctgtcactgtcgtggtgaccacggttttgctctgctcctttacagagatgatgtccacactgccgcctgtggagggtgtggaaagcttggtcactgttgtagtggtggttgtgacagtggattttgcacaattttctgtggaagaaaccacagtttgcttatcgcctttttctaccttgatcacagtttttgattctgtggccactgtggaggtcatcgtggtgacttctgtgatgacggtttttcttttagattctccattgacattttcatttttgttgatgggcagaccattttcatcaataaagtcattactgagattagattcctcttcagaagtaataggtgatgaagtaactttcttaacttctgaggtttctatttccatatcttctacctgattaactgaattgctttctggacaagatgctgagggtgtggtcgtctgtgtactgtcagactctttggttgatggcagggtctcaaggctatctcggtagttaccttcagcatctgaagaactcagcaaatgcgattttgtttcggagctgtttctttcattaaaatcttccatgatgacatcaccattaatgaatggccttatagcagattctttaacagtcaatgatttaatatcattctcagggattattttatttatattattaacctttggttcaacattaccacttactactctactctcagaaatttctttcaagcattcacctttcaaatatattttgggtttattatcttttccatttatttgaaatgtacttgttctctgtcctttcttttcagactctcgattttcattattctttttgtcagtggtattttttagctttatttgatcactacatttattaactggtctctcctctaatttcttctgctgacttggttttttaccatttgcttcagtccccttgaccggcagcctgtcctcacagtttccagtggactcaccagaaaccaactcacactttaacggctccaagacttcaacatcttgttctcgagttctgaactgttcagaaatgctttcattgctattctgaacaatcatatcttcttcactgctatcctgaatagacacggtatcagaactattttccaaagtgctattagattcagagtcacatcccagttttccttcaaagtccattgctcttgacagaggtgtggcatctctgtcattggtacttttaggcactgatgaatgtaaagcactcttggaagaagaaacaatggtgtcactttcctcctgtatgagcggttttttgttcttacagatcaaagtaccaatatcatctgcactggctagtttagagtcatcgatgaaaaaatcatttccttttgttttactcttactgggttcctggcctctactggcaaggtcagagactttttcttctatgtcattttcaatggaattttgtttcggacattttgtttctgggctccgaatggagacatcatctaacactcgatcttttggataaagtttgtttgtggtatgactaggatcactcattctaagaactgaggaatcactttctgaacatccctgaatcaagtcctcaggttgatcattatttgcatttgggctctgttcttgtctcatcgagtcactctgacacccttcttttgctttcgttattactggtgattcagagagattttttgaagaatttgtagaagtctttcctatacccttaattccaccctccaacttgattttttcgagtcgctgtttttcttccagtgtaaactgtttaattctcctttcaagaagtccatctagtttggatgattttgttttctttttgtaactagtccttagatgaaaaccctcactaacattgaccacatctacttgagaactctcctgacaatttacatgtgactctgttttcatgtcatcgtctacttccattggttcttccttgcagggtttatcactgtcagaatctaagagctccttcacatcttggtccttcttctcagtaatctttgagatatccatttcattttggtctgctccttttgcagcatctgaaccttttacctcatctttttcagaatcaggctctatttttattttttttggacttcgtgaacattttcttttatctgactcatccatattttcatccatattatttttggttccttctaacgactttctgtaattcacattagtattgcctggcaatttaggaacaaacctataaacatgagttttactaatccagctccaaccaccatatcctgtcactctgtactcttcacctttttgtttccaaacctgatgcttaactggaaatgtgtattttacccatgtcgcttgctgcatcgtttcttcttcttcctgtttcttctctttttttttgactttctccttttcttctctttcaattgatgtcatccggtgtaacctggtatgtcctaaagattctcgccatattggtagcatcacaactggtttaactgcacactccaaaatggctaaagccaatgcaaattctctgggtttgctacacatctgaactgccttgatccaatttgccctatgtgatgcccagttgggatgaagaaaggatgaagggatgttgttttctaattgggtgatagtcagtctcagagtagatatggtaagaactttggacccatggacagaaccgttccatttgaactctcctgctggagtcagacagaacttatgtgcaagatgccttctcttatcatggtcttctctgtgctggtgcttattcaaagcaaatgaattggtggagtattgattgtggtagacgcgatacttcccttcttgacccaatttaaaataattgttgatatttcctttcatgatcacttcctttttggtgctcaaccgtgaaatttctccttgagagttaactaccagtacctctttgccctccttaaataatttatttgcttcatgtgcagcggctgccacctgctggctcttcagctgactaagtttgctatctggattccgcaatctggtgatgattcgagttgagccagatgctccttttccagctccaggagattcacttagctccccgttggacttctccgatttgaaatcacctactatctcttcctgaatagagacaggtgtatgagattctctttctccattttcaggatcatcagctgccttagcagattcactctgggaagaatttagttcactgctgctgttactgttttccagattaggctggatggaggtagtggtagcactagtgttactgctctcacatgtcttgttaggttcttctggcacatcctgggggagctcagatgccaccttcttctctgccatgttgctgctatcgggggtttctgagagacaccccacagggctcctcccttcagagggactagtctcttctgaagttgcatttgttgtgttgtcgccaagatttgctgacacagagttacctttatccccaacttctgttggctcctcagattttccttgctcagggtcatcatctggtgttttgtcgtcactgtctttttcaagggactggtcttcaaattcttctctgtttttctcagcatctttagagtcattctcagtctcattcttgtctttttctgtttcttctgggcttttaacattatcaatgtctccctttttggctcttatggattccaaaatttcttcattagctgccgccagaaaggatttgttactgccccgagccttattggtcaggtcttcagttatgtccatgtgtcggtggatttcttcacgcatttcttctagaattttgcagagttctgcttcccaataatctttgtctagacagtcaattaattctgcaagttggacctttgtgctgtaataccaaattttcttttcattttcattttctgtatcttcttctattatgagtcttcggttcaagaaccagtatttcctccgacttctatcatatccaataggttcatgtcgaatatatggtttatttttttggatttcagcaacacagtcagtcacaccaggcaccttgtgtgctacacagacttcacactgccactcgtcctctggcacctcctcaagaggtggcttcacacattccaaatggtatactgctgaacatgtctcacagcaaagcaaatccccaagtttgtgacaaaccctacaatggtcatcatactgtatcaccccttcagacatcaattcctctcgagcaatatttgttgtaagaaactgatcgactagaaactgtagaactttgatcttgttctctactggtccatatgggtagtcctctgcctcttggtaaggaagaacgtgatggtactccttatcactctcacagtacacccgcagcacctctggccacgtcatcccatctatgaaatacagtgtggaattaacgctatctttcagatcagcaggtccaaaggtagtattggaagtgtcttcttcacgcagaactgctttcaaaagcacaacatgcatctctgccatgagtgtgcactgctcttggctcaccagagctgcacaaaagtcctcaaagcgaaaaggagataatctcaaaacagtgccaaagttccgcagtacctcgtaaatggcaatgacattcattatatgctcattaggcaccattaaatcctcagaggacttgggaaattcaaggggcgggatgtctttttcttccaatataggagaacgaggccgatgtactcttggttttcgcctacctggagtgctgctgtaggtactatggctcctgaagctgctttccgtgcagtaactggcgtcgtcgtcgtcgtcttccatctcctccggataatcggagtcatcgtcgtcctcttccatctcatcctcctcgtcgtcctcagaatcctgggtctcctcggcgtcgccgtcctcctcctcctcctcctcggagaccatgtcctcctcttcctcctcctcctcgctctcgtggtcatcgtacaccactttgttgacggccctccgggccgcggtggtccgggccaggtggccgccgccgcccccgccccccgtcctgccgcccccgcctcctcgccccccccggcccggggcgctggtgctggggggggccggcggcggcggcggcggcttcctccggctactgctgccccccctgggcgagctcagccgcgtcttgggcgccacctcagcctgggcggcggcccacctgccccggctgctgccgcggtgccgcgagcggagccccccgatgggtccggacgtgggcggcggcggcggtggcggcggggccggggcgcagcgctccgcagcgggagccgcgggctgcttgggcggcctgccccgccggcccctcatgtcggagccgaggcggggggagaaggaaagcgaagggggaggggcgggcgcagggggggcggtggggagcgccggggccgggtggggaggcccgcggggccgggcgggaggggcccggccgacggaagcgggtggagggagaaggctcaatccgaattgctggggccccactccggatcgccttcagccgccatcttgtttcttccct

SEQ ID NO: 9375 - RNA, 208 nt, Homo sapiens
  source 1..208: mol_type = other RNA
aggaagccctggaggggctggaggtgaggggcacgcccgctcaactgcactgcagccgctgcaaatccaaggctgccacaccccccggcagccagggacacggcttcatcttcctctttctccagcggaaagggggccctctccacggaacgccccacctgctagagtcctccacatcccgaaacgcaacgcccgagagcaggcgcgg

SEQ ID NO: 9376 - RNA, 80 nt, Homo sapiens
  source 1..80: mol_type = other RNA
aggaccttccctgaaccaaggaagagactgtgactcttccttggttcagggaaggtcctgaaccaaatcgagggtcggta

SEQ ID NO: 9377 - RNA, 751 nt, Homo sapiens
  source 1..751: mol_type = other RNA
aggactggactcccggcagcccgaggaaggagagtgatgcggaaagcgtctacggagcccggactgctggggcagctcgcggcagcattgcggctgcactgggcagcccccccgggaacttcccgcctacgaccgagctcgttcaggctttctgctgtaggcactcattgagctgctgccgccgctgtcctttccttcctttcccggttttgtgggggcctctggagatggggagagtcctgggaaacgtaggccaagttctgagtagggagagtcgccgcagttccggggcagccagtccggtcgccgtctcggcgagcgctcagcagcctcggcgcccggtgccactttgccacctctcgcggtccccggcctgtgcccctttgctgcggacagggcagccgccagccagctgtgccctggagcagagcctggcagcactgcttcctccttggccgcaccgctcccagtgacagtttcttttgtagctgatccccccctagatcgccggtccctgctcctttcacccctacaggcacttgcgtgtcgcccccttttttgcttttttccttcactccctcccttgctgcttttttcgctgaaacaattgctgcttctgttgcctctcagagagggtgccggtttcttctcccttttttccgacctcatcagctttttttgaaaagaaaaaaattgagcgctttttgagttgaaaaacccgcccccattttaacggcagagttttaaggag

SEQ ID NO: 9378 - RNA, 2099 nt, Homo sapiens
  source 1..2099: mol_type = other RNA
aggagaagtaaagtagaatctgatgagagagacttgggaacagagaggaagccaactgccttgccaatttcactactgccatcattattttctttatccatttctttttcatcttttgtttctatttcttcactactaagaaggaattctgcagtctcctgatttccttcttcttcctcctcctcttctttctcctcctcttcctctagttcttcctctttctcttctttctctaccttctcttctccatcttcctcagactcatctgtcatttcttcctcttcctcctcctcttcctcaaacccatcttcattatctaatttaaacagtgcttggcgcttctggcgctcctcaaaccttcggagtttcattgcttcttgcagtttagcttttaacacctgaagcttttcacctctgttggtttcaggttcaagtatcacaaaggaatcttcatcagcacctagccgtggtttaatggaaacatctactcccagttgcttaagtctatccagagtaaaccgtctcactttttcaggtggcccaactgctgatgatttattttgctgctcaggctcttccactttctcatctgtttcttctggattttgggggccttcaccctccagggcatgaggttcaaatgctacaagccctccaacctgacattcctcactgtgattgttcccgaggaagttggattcctgttgcaacactgagctgtccccaggtgaaggtctaatgtcactctgcttctgtttctcctgaatttctagctcttcattttttaccaaatccttcctgcaagactcatctgatccagtaatgatctgggtttcctttgaaactacagggagtgcattagtttccacttcattttctgcacctgttgtctgctcagaacctttactatggtgatcactgttcatttcagtagtatttgcagtgtctatgatttctttgtgatggcttgactgatatttagatgacttcaatagtgccatggcatttccgtggcaagtgggccggggtttacgtttgaagaaatcatgaatggttttattctcaggcatatgatatggaaggttcagtgcagactctcgaataaggcgctgagtctcactatgcagttgttttaatgcttctttacttaatctggctgcctttctttccttcctcgtggttccttttgataactcacttccttcctcaaatgaatggaccccactctccaaagatggttcttttttcttgtgcttttttactttgttttttacagctgctcttattgattctaatgactcttcatcttccaatggagagttattttcatcctccaacccagtttcaaaaaggtctttatccacaagaagacagccactgtcattaaatggctgttctacatcatcttcctggttttttgtttccttcttttttagctgtctaattttttccatttttctctcctctttctcaagtcttctttttgattttacttttgcttttcctgcagttccttctttatcatgtatgtgctttttggaactctttctgtcagtggtaaagtctgtagagtttccagactgaagactcagctctaagcaaggtttcacttgcgcttcaagattttcctgatacaaagacttttccatgtaactttcatcactgtctgccacagttttgtaaatccttttgatttttgtatttttcccagcatataaattctctttattttcctcctcggcactgtcataggtagttttctctggagaggcatttgtgtcctctgtttcggaatcactgtcttgtagaaccttcctgtttttcaacttcttacttacaaatatctcttcatctgaatctccttcactcaagggtccaattgtttcatagctgccctgtccactatctgaaggactatctgcttcctcttgtgaaatgacgtttgggtcattgatttctaggtgaacctcagaacccacctcgcctgtcatgacttctgcctcccctgcgctccactagggacggagctgtctctgattccctcagccggagagcagcggctcccgccgtctccagcccagcagtgctgttcttgcttt

SEQ ID NO: 9379 - RNA, 2129 nt, Homo sapiens
  source 1..2129: mol_type = other RNA
aggagaagtaaagtagaatctgatgagagagacttgggaacagagaggaagccaactgccttgccaatttcactactgccatcattattttctttatccatttctttttcatcttttgtttctatttcttcactactaagaaggaattctgcagtctcctgatttccttcttcttcctcctcctcttctttctcctcctcttcctctagttcttcctctttctcttctttctctaccttctcttctccatcttcctcagactcatctgtcatttcttcctcttcctcctcctcttcctcaaacccatcttcattatctaatttaaacagtgcttggcgcttctggcgctcctcaaaccttcggagtttcattgcttcttgcagtttagcttttaacacctgaagcttttcacctggttttgtgtggcttgctccatccaacttcttaggtgctaaagtcacaggtaccacatctgcttttagctcttcctttccatcagtgcccatgtctttcactatgacgttcacattcactgtctgaccagccctgggtttggctgctggattagcatgcttccagaaacgctgcttcaaggcttccagttctctgttggtttcaggttcaagtatcacaaaggaatcttcatcagcacctagccgtggtttaatggaaacatctactcccagttgcttaagtctatccagagtaaaccgtctcactttttcaggtggcccaactgctgatgatttattttgctgctcaggctcttccactttctcatctgtttcttctggattttgggggccttcaccctccagggcatgaggttcaaatgctacaagccctccaacctgacattcctcactgtgattgttcccgaggaagttggattcctgttgcaacactgagctgtccccaggtgaaggtctaatgtcactctgcttctgtttctcctgaatttctagctcttcattttttaccaaatccttcctgcaagactcatctgatccagtaatgatctgggtttcctttgaaactacagggagtgcattagtttccacttcattttctgcacctgttgtctgctcagaacctttactatggtgatcactgttcatttcagtagtatttgcagtgtctatgatttctttgtgatggcttgactgatatttagatgacttcaatagtgccatggcatttccgtggcaagtgggccggggtttacgtttgaagaaatcatgaatggttttattctcaggcatatgatatggaaggttcagtgcagactctcgaataaggcgctgagtctcactatgcagttgttttaatgcttctttacttaatctggctgcctttctttccttcctcgtggttccttttgataactcacttccttcctcaaatgaatggaccccactctccaaagatggttcttttttctggttttttgtttccttcttttttagctgtctaattttttccatttttctctcctctttctcaagtcttctttttgattttacttttgcttttcctgcagttccttctttatcatgtatgtgctttttggaactctttctgtcagtggtaaagtctgtagagtttccagactgaagactcagctctaagcaaggtttcacttgcgcttcaagattttcctgatacaaagacttttccatgtaactttcatcactgtctgccacagttttgtaaatccttttgatttttgtatttttcccagcatataaattctctttattttcctcctcggcactgtcataggtagttttctctggagaggcatttgtgtcctctgtttcggaatcactgtcttgtagaaccttcctgtttttcaacttcttacttacaaatatctcttcatctgaatctccttcactcaagggtccaattgtttcatagctgccctgtccactatctgaaggactatctgcttcctcttgtgaaatgacgtttgggtcattgatttctaggtgaacctcagaacccacctcgcctgtcatgacttctgcctcccctgcgctccactagggacggagctgtctctgattccctcagccggagagcagcggctcccgccgtctccagcccagcagtgctgttcttgcttt

SEQ ID NO: 9380 - RNA, 2291 nt, Homo sapiens
  source 1..2291: mol_type = other RNA
aggagaagtaaagtagaatctgatgagagagacttgggaacagagaggaagccaactgccttgccaatttcactactgccatcattattttctttatccatttctttttcatcttttgtttctatttcttcactactaagaaggaattctgcagtctcctgatttccttcttcttcctcctcctcttctttctcctcctcttcctctagttcttcctctttctcttctttctctaccttctcttctccatcttcctcagactcatctgtcatttcttcctcttcctcctcctcttcctcaaacccatcttcattatctaatttaaacagtgcttggcgcttctggcgctcctcaaaccttcggagtttcattgcttcttgcagtttagcttttaacacctgaagcttttcacctggttttgtgtggcttgctccatccaacttcttaggtgctaaagtcacaggtaccacatctgcttttagctcttcctttccatcagtgcccatgtctttcactatgacgttcacattcactgtctgaccagccctgggtttggctgctggattagcatgcttccagaaacgctgcttcaaggcttccagttctctgttggtttcaggttcaagtatcacaaaggaatcttcatcagcacctagccgtggtttaatggaaacatctactcccagttgcttaagtctatccagagtaaaccgtctcactttttcaggtggcccaactgctgatgatttattttgctgctcaggctcttccactttctcatctgtttcttctggattttgggggccttcaccctccagggcatgaggttcaaatgctacaagccctccaacctgacattcctcactgtgattgttcccgaggaagttggattcctgttgcaacactgagctgtccccaggtgaaggtctaatgtcactctgcttctgtttctcctgaatttctagctcttcattttttaccaaatccttcctgcaagactcatctgatccagtaatgatctgggtttcctttgaaactacagggagtgcattagtttccacttcattttctgcacctgttgtctgctcagaacctttactatggtgatcactgttcatttcagtagtatttgcagtgtctatgatttctttgtgatggcttgactgatatttagatgacttcaatagtgccatggcatttccgtggcaagtgggccggggtttacgtttgaagaaatcatgaatggttttattctcaggcatatgatatggaaggttcagtgcagactctcgaataaggcgctgagtctcactatgcagttgttttaatgcttctttacttaatctggctgcctttctttccttcctcgtggttccttttgataactcacttccttcctcaaatgaatggaccccactctccaaagatggttcttttttcttgtgcttttttactttgttttttacagctgctcttattgattctaatgactcttcatcttccaatggagagttattttcatcctccaacccagtttcaaaaaggtctttatccacaagaagacagccactgtcattaaatggctgttctacatcatcttcctggttttttgtttccttcttttttagctgtctaattttttccatttttctctcctctttctcaagtcttctttttgattttacttttgcttttcctgcagttccttctttatcatgtatgtgctttttggaactctttctgtcagtggtaaagtctgtagagtttccagactgaagactcagctctaagcaaggtttcacttgcgcttcaagattttcctgatacaaagacttttccatgtaactttcatcactgtctgccacagttttgtaaatccttttgatttttgtatttttcccagcatataaattctctttattttcctcctcggcactgtcataggtagttttctctggagaggcatttgtgtcctctgtttcggaatcactgtcttgtagaaccttcctgtttttcaacttcttacttacaaatatctcttcatctgaatctccttcactcaagggtccaattgtttcatagctgccctgtccactatctgaaggactatctgcttcctcttgtgaaatgacgtttgggtcattgatttctaggtgaacctcagaacccacctcgcctgtcatgacttctgcctcccctgcgctccactagggacggagctgtctctgattccctcagccggagagcagcggctcccgccgtctccagcccagcagtgctgttcttgcttt

SEQ ID NO: 9381 - RNA, 2286 nt, Homo sapiens
  source 1..2286: mol_type = other RNA
aggagaagtaaagtagaatctgatgagagagacttgggaacagagaggaagccaactgccttgccaatttcactactgccatcattattttctttatccatttctttttcatcttttgtttctatttcttcactactaagaaggaattctgcagtctcctgatttccttcttcttcctcctcctcttctttctcctcctcttcctctagttcttcctctttctcttctttctctaccttctcttctccatcttcctcagactcatctgtcatttcttcctcttcctcctcctcttcctcaaacccatcttcattatctaatttaaacagtgcttggcgcttctggcgctcctcaaaccttcggagtttcattgcttcttgcagtttagcttttaacacctgaagcttttcacctggttttgtgtggcttgctccatccaacttcttaggtgctaaagtcacaggtaccacatctgcttttagctcttcctttccatcagtgcccatgtctttcactatgacgttcacattcactgtctgaccagccctgggtttggctgctggattagcatgcttccagaaacgctgcttcaaggcttccagttctctgttggtttcaggttcaagtatcacaaaggaatcttcatcagcacctagccgtggtttaatggaaacatctactcccagttgcttaagtctatccagagtaaaccgtctcactttttcaggtggcccaactgctgatgatttattttgctgctcaggctcttccactttctcatctgtttcttctggattttgggggccttcaccctccagggcatgaggttcaaatgctacaagccctccaacctgacattcctcactgtgattgttcccgaggaagttggattcctgttgcaacactgagctgtccccaggtgaaggtctaatgtcactctgcttctgtttctcctgaatttctagctcttcattttttaccaaatccttcctgcaagactcatctgatccagtaatgatctgggtttcctttgaaactacagggagtgcattagtttccacttcattttctgcacctgttgtctgctcagaacctttactatggtgatcactgttcatttcagtagtatttgcagtgtctatgatttctttgtgatggcttgactgatatttagatgacttcaatagtgccatggcatttccgtggcaagtgggccggggtttacgtttgaagaaatcatgaatggttttattctcaggcatatgatatggaaggttcagtgcagactctcgaataaggcgctgagtctcactatgcagttgttttaatgcttctttacttaatctggctgcctttctttccttcctcgtggttccttttgataactcacttccttcctcaaatgaatggaccccactctccaaagatggttcttttttcttgtgcttttttactttgttttttacagctgctcttattgattctaatgactcttcatcttccaatggagagttattttcatcctccaacccagtttcaaaaaggtctttatccacaagaagacagccactgtcattaaatggctgttctacatcatcttcctggttttttgtttccttcttttttagctgtctaattttttccatttttctctcctctttctcaagtcttctttttgattttacttttgcttttcctgcagttccttctttatcatgtatgtgctttttggaactctttctgtcagtggtaaagtctgtagagtttccagactgaagactcagctctaagcaaggtttcacttgcgcttcaagattttcctgatacaaagacttttccatgtaactttcatcactgtctgccacagttttgtaaatccttttgatttttgtatttttcccagcatataaattctctttattttcctcctcggcactgtcataggtagttttctctggagaggcatttgtgtcctctgtttcggaatcactgtcttgtagaaccttcctgtttttcaacttcttacttacaaatatctcttcatctgaatctccttcactcaagggtccaattgtttcatagctgccctgtccactatctgaaggactatctgcttcctcttgtgaaatgacgtttgggtcattgatttctaggtgaacctcgcctgtcatgacttctgcctcccctgcgctccactagggacggagctgtctctgattccctcagccggagagcagcggctcccgccgtctccagcccagcagtgctgttcttgctttcccgccc

SEQ ID NO: 9382 - RNA, 3871 nt, Homo sapiens
  source 1..3871: mol_type = other RNA
aggagagtggattccaggtggtaagaaacaaacccaactgaaactggcttaagggaggctacagggatatattgaccccaaccacacatctacagaaacagacttaacggtgtcacgaggccccatccttctccctctgaggccagctctccctgactgctgggaaacagctcccaggaggtccaggcgtatcctaccagcttagtcagtccaggaatgggaaacagcacctctgcttgcccagccccagggaagatcatagagggctcccactgacctgcatgcacctgtgacaattgctgtggccagagaactccggtgctgcagccagacctggatgctatgcccagccttggaactaaagaactgtgaggtcagtgacccagtcccatggcctgagggtgtgtgcctttgcagagctctcaggttcctcgggggctgtcccctccaccagcctcagggccctggctcagaagccacaccctcagcctcatcccagggtatgttcagtgttggcccttgtggcccctgccggcacacacttggaactgggccaggcaccccagggcctgagcgtgtggctgaacatttgaccagtgaggaatcaggaactgcccagaggagtgacacccacccccagcccagggctctgcccagagggaaagtgggggagccctagtgtaacccctcctggctggctgtggcttgggccctgtatgtccccatctctgcccaacttccctgtcctcatcagggggctgatgcagtggcttcagtgtcagtgactaaccagtggccctggagtgactcgtaaggcaggtaccctgtggacagttatttgtctgggggaggttagtgccacccactccagctggctgaggtgccagcgaggtctaacccattacgttgagaatggagccaccctaggggtggagcagcttgctgaggtcaccgaggtcatcctcagaaatgccagcccctgccctactcacagaggggcaagctagggcatggggacaaggactgggattccctgaggcctgggcgctccatgttgcctgagtcaacctggcccatccacctgtcatctctgcagcctcacccaccacccccgcagcctctcctgccacagagatgccagatgaggaggccagcatggtgcagaggagtaagtgggcttagcaggatggggcaggccctgtggcaggacggggcaggcctggtccctggtcagatcaggatgcggagagcaactccgggctctcaacacctccatttattgcatgtataccctgacttcctcactggtccttctgtgcctgctctcatgctggcaccggcttgtggccgcactccttggaagctatgtccacggctctggctcaggttcacctgggggtgtgggcctcacagggctcattcggaccctgggttgcggccccagtccagccccctattctcccatctgggcagatggaggaacccttgcctcctgctgcccgccaagtcctccatttaaggcccacctgggctggattgccctggacggaagagcgcacaggccaccggccatagcttgcccctgtgggccaagtccccagtgtggtggccttcgccggcttgccctgaggcacggcccgacgggggcgccctggaggcgctgttggcccggtgggcagcgtggggggtatcgcgggtaggggacttgggcgggctgggcggcttgagcgcgctgacggctcggatgagacccatgcgccggcggatggagtggtccaggttgaccgtgcagcgcagcaggctctgcgcctcggccacggtgaaggggaagtcggcgcccaggaagcgctcgaagagctcggggtcgccgtccaggtcgagcacgttctgcaacgccttggtcatggtgtgcagctcgcggctgttgtcgcggaaaacgtcccagaggcgcgcgcggccctcgggcgcgcccccggtctgctgccggtcctccaggcactgcagcgcccagctcaggcggcacggccactggttggcgagcaccacccacgccaccgcctggcgcggcgtggggcccccaaagtccccctgctgctgctgctgctgcagcaggcgcacggtgatgggcacggtgttgacgatgcgccgcatggacaccacgttgtcgggcacgtactcgtagaggcagtcgcgctcgtcgtgaaggcagaagagcgcctcctggattcgccgcgccgcctcgtcgtcgatgcggccctgcccgcgctccgtccccgcctgcgcctgcaccgccagcagctgcgcgctctcgcccccggcgtcccccggcagccacggcttgcgcgtcatctcgcggtacaacaggtcgtcgcggctctgcaccgcatcgtgcaggaactgcagcttggtgcggcggcccataatgggcacagagaagggcagcgtgacagtgcggttgaggaagaggtagccgttatcggccgtgcccttcatgttgcccgcgctctctaggcacgcggccaggatgctggggtccacgaccaggatgaagatgaagggcgcgtggctgtcggacagcagcgtgttgatggcgttgagcacgcccaccacgcgctccgggtagcacgtgtccagcccggtgacctccagcaccacgcgcagcctgcgccgctggtagatctccaggaagcacaggaagtcggtgagcagctccacctccttcttcacctcgcacatgaaacccagctggctgccgaacttttcacgcgacaccagccgctcgatcttcttgcgctggcttacgaacaggtgcttgcccaccgagtacacggccatgagcagccccgagcccgacagtgtggtggccgcgccgccaaacaccttgagcaggctgccgctcgggctgccgtggcccagcgcgtggccgcccagtgacaagtagagcagccccacacccaggcccagcgccgccagcagcgccagcagccccaggcacacgcggcgccgacaatgccactcgctctggcagcagtcctgcctggtggccggcttgttgcccagcaccgagtacacgctgaagggcagtgcgccatagtggcggcggatgccctcgcacaacgtggtcaccaggccggcccacagcttgtcggtgcccgcgtactgccaggcgctaaagcggatgaaaaggaactgcacgttcctgcgccgcaggtgcacctcggtgatgatgggctgcaggaacaccaggtaccacagtagctgcgggacgccccagccgctcacggcacgcggccgccactgcacgtgctgcagctcctcgctctcgcgctgcgcggcctcctgctgcatcagcgccgtgatcttgtccagcatcatgtgcaggcggcagccgaaaggggcatagaaacccacggtcacagggaccggcacgtggcagagtgtcttggccaggcagctgcagtagacgtcatcctctgtcaggatgtccatgtcaggcagcgggcggcgaagcccaggagtccccagatgctacagatgcgagcggggtgggagggggcagcataagggccactctgcccagggacgggcagcaggagtgcgtaggggccgcgtgtgtccatgggggtgtctggcctccccctaccccatgcatccccagccctggcagccccagcccgacctggcctacactccgggcactcccagccctgctccccaggaagacgctccgttctgtgcacatcgccgggcagagggcagccccagacttgttgacttggcagaggtgccagtaaggccgcccatgccggaggccagcatccctctgccaggagcacggggagggagggagtggagggggacgtggcagggg

SEQ ID NO: 9383 - RNA, 4014 nt, Homo sapiens
  source 1..4014: mol_type = other RNA
aggagagtggattccaggtggtaagaaacaaacccaactgaaactggcttaagggaggctacagggatatattgaccccaaccacacatctacagaaacagacttaacggtgtcacgaggccccatccttctccctctgaggccagctctccctgactgctgggaaacagctcccaggaggtccaggcgtatcctaccagcttagtcagtccaggaatgggaaacagcacctctgcttgcccagccccagggaagatcatagagggctcccactgacctgcatgcacctgtgacaattgctgtggccagagaactccggtgctgcagccagacctggatgctatgcccagccttggaactaaagaactgtgaggtcagtgacccagtcccatggcctgagggtgtgtgcctttgcagagctctcaggttcctcgggggctgtcccctccaccagcctcagggccctggctcagaagccacaccctcagcctcatcccagggtatgttcagtgttggcccttgtggcccctgccggcacacacttggaactgggccaggcaccccagggcctgagcgtgtggctgaacatttgaccagtgaggaatcaggaactgcccagaggagtgacacccacccccagcccagggctctgcccagagggaaagtgggggagccctagtgtaacccctcctggctggctgtggcttgggccctgtatgtccccatctctgcccaacttccctgtcctcatcagggggctgatgcagtggcttcagtgtcagtgactaaccagtggccctggagtgactcgtaaggcaggtaccctgtggacagttatttgtctgggggaggttagtgccacccactccagctggctgaggtgccagcgaggtctaacccattacgttgagaatggagccaccctaggggtggagcagcttgctgaggtcaccgaggtcatcctcagaaatgccagcccctgccctactcacagaggggcaagctagggcatggggacaaggactgggattccctgaggcctgggcgctccatgttgcctgagtcaacctggcccatccacctgtcatctctgcagcctcacccaccacccccgcagcctctcctgccacagagatgccagatgaggaggccagcatggtgcagaggagtaagtgggcttagcaggatggggcaggccctgtggcaggacggggcaggcctggtccctggtcagatcaggatgcggagagcaactccgggctctcaacacctccatttattgcatgtataccctgacttcctcactggtccttctgtgcctgctctcatgctggcaccggcttgtggccgcactccttggaagctatgtccacggctctggctcaggttcacctgggggtgtgggcctcacagggctcattcggaccctgggttgcggccccagtccagccccctattctcccatctgggcagatggaggaacccttgcctcctgctgcccgccaagtcctccatttaaggcccacctgggctggattgccctggacggaagagcgcacaggccaccggccatagcttgcccctgtgggccaagtccccagtgtggtggccttcgccggcttgccctgaggcacggcccgacgggggcgccctggaggcgctgttggcccggtgggcagcgtggggggtatcgcgggtaggggacttgggcgggctgggcggcttgagcgcgctgacggctcggatgagacccatgcgccggcggatggagtggtccaggttgaccgtgcagcgcagcaggctctgcgcctcggccacggtgaaggggaagtcggcgcccaggaagcgctcgaagagctcggggtcgccgtccaggtcgagcacgttctgcaacgccttggtcatggtgtgcagctcgcggctgttgtcgcggaaaacgtcccagaggcgcgcgcggccctcgggcgcgcccccggtctgctgccggtcctccaggcactgcagcgcccagctcaggcggcacggccactggttggcgagcaccacccacgccaccgcctggcgcggcgtggggcccccaaagtccccctgctgctgctgctgctgcagcaggcgcacggtgatgggcacggtgttgacgatgcgccgcatggacaccacgttgtcgggcacgtactcgtagaggcagtcgcgctcgtcgtgaaggcagaagagcgcctcctggattcgccgcgccgcctcgtcgtcgatgcggccctgcccgcgctccgtccccgcctgcgcctgcaccgccagcagctgcgcgctctcgcccccggcgtcccccggcagccacggcttgcgcgtcatctcgcggtacaacaggtcgtcgcggctctgcaccgcatcgtgcaggaactgcagcttggtgcggcggcccataatgggcacagagaagggcagcgtgacagtgcggttgaggaagaggtagccgttatcggccgtgcccttcatgttgcccgcgctctctaggcacgcggccaggatgctggggtccacgaccaggatgaagatgaagggcgcgtggctgtcggacagcagcgtgttgatggcgttgagcacgcccaccacgcgctccgggtagcacgtgtccagcccggtgacctccagcaccacgcgcagcctgcgccgctggtagatctccaggaagcacaggaagtcggtgagcagctccacctccttcttcacctcgcacatgaaacccagctggctgccgaacttttcacgcgacaccagccgctcgatcttcttgcgctggcttacgaacaggtgcttgcccaccgagtacacggccatgagcagccccgagcccgacagtgtggtggccgcgccgccaaacaccttgagcaggctgccgctcgggctgccgtggcccagcgcgtggccgcccagtgacaagtagagcagccccacacccaggcccagcgccgccagcagcgccagcagccccaggcacacgcggcgccgacaatgccactcgctctggcagcagtcctgcctggtggccggcttgttgcccagcaccgagtacacgctgaagggcagtgcgccatagtggcggcggatgccctcgcacaacgtggtcaccaggccggcccacagcttgtcggtgcccgcgtactgccaggcgctaaagcggatgaaaaggaactgcacgttcctgcgccgcaggtgcacctcggtgatgatgggctgcaggaacaccaggtaccacagtagctgcgggacgccccagccgctcacggcacgcggccgccactgcacgtgctgcagctcctcgctctcgcgctgcgcggcctcctgctgcatcagcgccgtgatcttgtccagcatcatgtgcaggcggcagccgaaaggggcatagaaacccacggtcacagggaccggcacgtggcagagtgtcttggccaggcagctgcagtagacgtcatcctctgtcaggatgtcggagctgtaggcagtgaaggagccacaggccgctggggcgggcaggggccgggcatcagtgggctcgctgggcttcaggaggacgccagccgcggagggtagagctgggccactcctggccatggctggtgccgtggtgggtaaggtgggcgcctgaggggcgctggcaggttccttggggacagtggaggttgcaggcagccccttctgggcttcgtgaatggggcagagccgctgccgcagggggctgggaggtgagggctgggactggggctgccgctgctgctgcaggacggagggcaggaggccccggcgccagccactgccacccacttggtggctgtggtaggccagctgccagtgtgattggggggaaggccgacagggcccatgggctcggagggccgctgagtcctggcgccactgatgacagcatccttttcggtgccccaactctgggtcccagaagtagtgcccgttggggctctgggcatccttggcgaagtggactttgtaatgtttgtgcat

SEQ ID NO: 9384 - RNA, 5992 nt, Homo sapiens
  source 1..5992: mol_type = other RNA
aggagagtggattccaggtggtaagaaacaaacccaactgaaactggcttaagggaggctacagggatatattgaccccaaccacacatctacagaaacagacttaacggtgtcacgaggccccatccttctccctctgaggccagctctccctgactgctgggaaacagctcccaggaggtccaggcgtatcctaccagcttagtcagtccaggaatgggaaacagcacctctgcttgcccagccccagggaagatcatagagggctcccactgacctgcatgcacctgtgacaattgctgtggccagagaactccggtgctgcagccagacctggatgctatgcccagccttggaactaaagaactgtgaggtcagtgacccagtcccatggcctgagggtgtgtgcctttgcagagctctcaggttcctcgggggctgtcccctccaccagcctcagggccctggctcagaagccacaccctcagcctcatcccagggtatgttcagtgttggcccttgtggcccctgccggcacacacttggaactgggccaggcaccccagggcctgagcgtgtggctgaacatttgaccagtgaggaatcaggaactgcccagaggagtgacacccacccccagcccagggctctgcccagagggaaagtgggggagccctagtgtaacccctcctggctggctgtggcttgggccctgtatgtccccatctctgcccaacttccctgtcctcatcagggggctgatgcagtggcttcagtgtcagtgactaaccagtggccctggagtgactcgtaaggcaggtaccctgtggacagttatttgtctgggggaggttagtgccacccactccagctggctgaggtgccagcgaggtctaacccattacgttgagaatggagccaccctaggggtggagcagcttgctgaggtcaccgaggtcatcctcagaaatgccagcccctgccctactcacagaggggcaagctagggcatggggacaaggactgggattccctgaggcctgggcgctccatgttgcctgagtcaacctggcccatccacctgtcatctctgcagcctcacccaccacccccgcagcctctcctgccacagagatgccagatgaggaggccagcatggtgcagaggagtaagtgggcttagcaggatggggcaggccctgtggcaggacggggcaggcctggtccctggtcagatcaggatgcggagagcaactccgggctctcaacacctccatttattgcatgtataccctgacttcctcactggtccttctgtgcctgctctcatgctggcaccggcttgtggccgcactccttggaagctatgtccacggctctggctcaggttcacctgggggtgtgggcctcacagggctcattcggaccctgggttgcggccccagtccagccccctattctcccatctgggcagatggaggaacccttgcctcctgctgcccgccaagtcctccatttaaggcccacctgggctggattgccctggacggaagagcgcacaggccaccggccatagcttgcccctgtgggccaagtccccagtgtggtggccttcgccggcttgccctgaggcacggcccgacgggggcgccctggaggcgctgttggcccggtgggcagcgtggggggtatcgcgggtaggggacttgggcgggctgggcggcttgagcgcgctgacggctcggatgagacccatgcgccggcggatggagtggtccaggttgaccgtgcagcgcagcaggctctgcgcctcggccacggtgaaggggaagtcggcgcccaggaagcgctcgaagagctcggggtcgccgtccaggtcgagcacgttctgcaacgccttggtcatggtgtgcagctcgcggctgttgtcgcggaaaacgtcccagaggcgcgcgcggccctcgggcgcgcccccggtctgctgccggtcctccaggcactgcagcgcccagctcaggcggcacggccactggttggcgagcaccacccacgccaccgcctggcgcggcgtggggcccccaaagtccccctgctgctgctgctgctgcagcaggcgcacggtgatgggcacggtgttgacgatgcgccgcatggacaccacgttgtcgggcacgtactcgtagaggcagtcgcgctcgtcgtgaaggcagaagagcgcctcctggattcgccgcgccgcctcgtcgtcgatgcggccctgcccgcgctccgtccccgcctgcgcctgcaccgccagcagctgcgcgctctcgcccccggcgtcccccggcagccacggcttgcgcgtcatctcgcggtacaacaggtcgtcgcggctctgcaccgcatcgtgcaggaactgcagcttggtgcggcggcccataatgggcacagagaagggcagcgtgacagtgcggttgaggaagaggtagccgttatcggccgtgcccttcatgttgcccgcgctctctaggcacgcggccaggatgctggggtccacgaccaggatgaagatgaagggcgcgtggctgtcggacagcagcgtgttgatggcgttgagcacgcccaccacgcgctccgggtagcacgtgtccagcccggtgacctccagcaccacgcgcagcctgcgccgctggtagatctccaggaagcacaggaagtcggtgagcagctccacctccttcttcacctcgcacatgaaacccagctggctgccgaacttttcacgcgacaccagccgctcgatcttcttgcgctggcttacgaacaggtgcttgcccaccgagtacacggccatgagcagccccgagcccgacagtgtggtggccgcgccgccaaacaccttgagcaggctgccgctcgggctgccgtggcccagcgcgtggccgcccagtgacaagtagagcagccccacacccaggcccagcgccgccagcagcgccagcagccccaggcacacgcggcgccgacaatgccactcgctctggcagcagtcctgcctggtggccggcttgttgcccagcaccgagtacacgctgaagggcagtgcgccatagtggcggcggatgccctcgcacaacgtggtcaccaggccggcccacagcttgtcggtgcccgcgtactgccaggcgctaaagcggatgaaaaggaactgcacgttcctgcgccgcaggtgcacctcggtgatgatgggctgcaggaacaccaggtaccacagtagctgcgggacgccccagccgctcacggcacgcggccgccactgcacgtgctgcagctcctcgctctcgcgctgcgcggcctcctgctgcatcagcgccgtgatcttgtccagcatcatgtgcaggcggcagccgaaaggggcatagaaacccacggtcacagggaccggcacgtggcagagtgtcttggccaggcagctgcagtagacgtcatcctctgtcaggatgtcggagctgtaggcagtgaaggagccacaggccgctggggcgggcaggggccgggcatcagtgggctcgctgggcttcaggaggacgccagccgcggagggtagagctgggccactcctggccatggctggtgccgtggtgggtaaggtgggcgcctgaggggcgctggcaggttccttggggacagtggaggttgcaggcagccccttctgggcttcgtgaatggggcagagccgctgccgcagggggctgggaggtgagggctgggactggggctgccgctgctgctgcaggacggagggcaggaggccccggcgccagccactgccacccacttggtggctgtggtaggccagctgccagtgtgattggggggaaggccgacagggcccatgggctcggagggccgctgagtcctggcgccactgatgacagcatccttttcggtgccccaactctgggtcccagaagtagtgcccgttggggctctgggcatccttggcgaagtggactttgtaatgtttgtgcatggcagccgggcagctgggtgctgggggcctgctcctgaggcaggagggagcacacaggcttggcgtagcctctgacggtggcctcacggccccagctgcctgccccacgagcagctgccacaccagcccggactgtcagcgcaggcccatccagatggaggcctcagcccagtgcccgcctgaccggtttgcctgcctgtccccgccccttccccagcgcctgcctgtcccagtgctctctgctctcgaggactgggactccgactggactcagtcttgtgtccccatccctggtaaggaacggagatgcatcccgcagcactgcctcaatctccttaaggcagccacaggcccaggcacttctgctggtgtgggggggacagggagctgggatgccagctcctccgtggcccaggtatgtgaccttgggcaggtgacttcactctccgagccatggcttcctcattgctgagtgggcacctgcctctcgtggctgtcgcgagggaggcactgggtgggagtcccctcagctcagggcctggcgcacctgacccggggctgtgctgacccatttacctggcgctgttctaaatggatgtccataggacaagggcaacagcacacacatcaaggcttgctacaccatagccccgtcttcctctccaccacccagggggccaggtgtgatgcccgcttcacagatgaggacactgaggcccagagaagtgaagtcctcggccccagggcacacagaggcagggcggggatttggaagcagtcagtggttgctactcccaggctcgccaaggctctgtctcctgccctcggggccagcactcagtgactgcctccccacagatgccctctgaggggtgagggccggggtaaggctgggcaggagatgccctgaaggcccctcggctctctggggccccggctccctgtggctgctggcgtaacggggtcaacagttgcttccctgacagacggggtgctccgatggggatgggggaggcagccccagaacagtgcccaggacaagataaagggaacccacccagccctgagttctgcccaggtgaccaaacactgctccctacggccagagccagggcccttcctgcgacctgggaccccgtctcctcccccacccttcaagccggttgctctgggaaggttcctccctggcccaccagggaggcggggctggcatctgagcgtgggcatctgcagtgggcctccgtgccaaccccccacacccccggcccgatcatgaagcgtggcccaatgtaaatgagccgtctccgcaggacgagattgccccgggctgggagcacagtggccaggaggctgctggacactagggggagcaggcgtttggggagtgggccaggcgggcagcactgcagaggcagacacaggacacagctacactcagccaggtggaataggaaggggtgacccaggcagggcctgacggggtgactggaccccactctacaggggaggttctttagcaaggggcccctttctcatcccatttggggttcacccccagccttggtgggcagctctgagcctggggcacttacccatgtcaggcagcgggcggcgaagcccaggagtccccagatgctacagatgcgagcggggtgggagggggcagcataagggccactctgcccagggacgggcagcaggagtgcgtaggggccgcgtgtgtccatgggggtgtctggcctccccctaccccatgcatccccagccctggcagccccagcccgacctggcctacactccgggcactcccagccctgctccccaggaagacgctccgttctgtgcacatcgccgggcagagggcagccccagacttgttgacttggcagaggtgccagtaaggccgcccatgccggaggccagcatccctctgccaggagcacggggagggagggagtggagggggacgtggcagggg

SEQ ID NO: 9385 - RNA, 6253 nt, Homo sapiens
  source 1..6253: mol_type = other RNA
aggagagtggattccaggtggtaagaaacaaacccaactgaaactggcttaagggaggctacagggatatattgaccccaaccacacatctacagaaacagacttaacggtgtcacgaggccccatccttctccctctgaggccagctctccctgactgctgggaaacagctcccaggaggtccaggcgtatcctaccagcttagtcagtccaggaatgggaaacagcacctctgcttgcccagccccagggaagatcatagagggctcccactgacctgcatgcacctgtgacaattgctgtggccagagaactccggtgctgcagccagacctggatgctatgcccagccttggaactaaagaactgtgaggtcagtgacccagtcccatggcctgagggtgtgtgcctttgcagagctctcaggttcctcgggggctgtcccctccaccagcctcagggccctggctcagaagccacaccctcagcctcatcccagggtatgttcagtgttggcccttgtggcccctgccggcacacacttggaactgggccaggcaccccagggcctgagcgtgtggctgaacatttgaccagtgaggaatcaggaactgcccagaggagtgacacccacccccagcccagggctctgcccagagggaaagtgggggagccctagtgtaacccctcctggctggctgtggcttgggccctgtatgtccccatctctgcccaacttccctgtcctcatcagggggctgatgcagtggcttcagtgtcagtgactaaccagtggccctggagtgactcgtaaggcaggtaccctgtggacagttatttgtctgggggaggttagtgccacccactccagctggctgaggtgccagcgaggtctaacccattacgttgagaatggagccaccctaggggtggagcagcttgctgaggtcaccgaggtcatcctcagaaatgccagcccctgccctactcacagaggggcaagctagggcatggggacaaggactgggattccctgaggcctgggcgctccatgttgcctgagtcaacctggcccatccacctgtcatctctgcagcctcacccaccacccccgcagcctctcctgccacagagatgccagatgaggaggccagcatggtgcagaggagtaagtgggcttagcaggatggggcaggccctgtggcaggacggggcaggcctggtccctggtcagatcaggatgcggagagcaactccgggctctcaacacctccatttattgcatgtataccctgacttcctcactggtccttctgtgcctgctctcatgctggcaccggcttgtggccgcactccttggaagctatgtccacggctctggctcaggttcacctgggggtgtgggcctcacagggctcattcggaccctgggttgcggccccagtccagccccctattctcccatctgggcagatggaggaacccttgcctcctgctgcccgccaagtcctccatttaaggcccacctgggctggattgccctggacggaagagcgcacaggccaccggccatagcttgcccctgtgggccaagtccccagtgtggtggccttcgccggcttgccctgaggcacggcccgacgggggcgccctggaggcgctgttggcccggtgggcagcgtggggggtatcgcgggtaggggacttgggcgggctgggcggcttgagcgcgctgacggctcggatgagacccatgcgccggcggatggagtggtccaggttgaccgtgcagcgcagcaggctctgcgcctcggccacggtgaaggggaagtcggcgcccaggaagcgctcgaagagctcggggtcgccgtccaggtcgagcacgttctgcaacgccttggtcatggtgtgcagctcgcggctgttgtcgcggaaaacgtcccagaggcgcgcgcggccctcgggcgcgcccccggtctgctgccggtcctccaggcactgcagcgcccagctcaggcggcacggccactggttggcgagcaccacccacgccaccgcctggcgcggcgtggggcccccaaagtccccctgctgctgctgctgctgcagcaggcgcacggtgatgggcacggtgttgacgatgcgccgcatggacaccacgttgtcgggcacgtactcgtagaggcagtcgcgctcgtcgtgaaggcagaagagcgcctcctggattcgccgcgccgcctcgtcgtcgatgcggccctgcccgcgctccgtccccgcctgcgcctgcaccgccagcagctgcgcgctctcgcccccggcgtcccccggcagccacggcttgcgcgtcatctcgcggtacaacaggtcgtcgcggctctgcaccgcatcgtgcaggaactgcagcttggtgcggcggcccataatgggcacagagaagggcagcgtgacagtgcggttgaggaagaggtagccgttatcggccgtgcccttcatgttgcccgcgctctctaggcacgcggccaggatgctggggtccacgaccaggatgaagatgaagggcgcgtggctgtcggacagcagcgtgttgatggcgttgagcacgcccaccacgcgctccgggtagcacgtgtccagcccggtgacctccagcaccacgcgcagcctgcgccgctggtagatctccaggaagcacaggaagtcggtgagcagctccacctccttcttcacctcgcacatgaaacccagctggctgccgaacttttcacgcgacaccagccgctcgatcttcttgcgctggcttacgaacaggtgcttgcccaccgagtacacggccatgagcagccccgagcccgacagtgtggtggccgcgccgccaaacaccttgagcaggctgccgctcgggctgccgtggcccagcgcgtggccgcccagtgacaagtagagcagccccacacccaggcccagcgccgccagcagcgccagcagccccaggcacacgcggcgccgacaatgccactcgctctggcagcagtcctgcctggtggccggcttgttgcccagcaccgagtacacgctgaagggcagtgcgccatagtggcggcggatgccctcgcacaacgtggtcaccaggccggcccacagcttgtcggtgcccgcgtactgccaggcgctaaagcggatgaaaaggaactgcacgttcctgcgccgcaggtgcacctcggtgatgatgggctgcaggaacaccaggtaccacagtagctgcgggacgccccagccgctcacggcacgcggccgccactgcacgtgctgcagctcctcgctctcgcgctgcgcggcctcctgctgcatcagcgccgtgatcttgtccagcatcatgtgcaggcggcagccgaaaggggcatagaaacccacggtcacagggaccggcacgtggcagagtgtcttggccaggcagctgcagtagacgtcatcctctgtcaggatgtcggagctgtaggcagtgaaggagccacaggccgctggggcgggcaggggccgggcatcagtgggctcgctgggcttcaggaggacgccagccgcggagggtagagctgggccactcctggccatggctggtgccgtggtgggtaaggtgggcgcctgaggggcgctggcaggttccttggggacagtggaggttgcaggcagccccttctgggcttcgtgaatggggcagagccgctgccgcagggggctgggaggtgagggctgggactggggctgccgctgctgctgcaggacggagggcaggaggccccggcgccagccactgccacccacttggtggctgtggtaggccagctgccagtgtgattggggggaaggccgacagggcccatgggctcggagggccgctgagtcctggcgccactgatgacagcatccttttcggtgccccaactctgggtcccagaagtagtgcccgttggggctctgggcatccttggcgaagtggactttgtaatgtttgtgcatggcagccgggcagctgggtgctgggggcctgctcctgaggcaggagggagcacacaggcttggcgtagcctctgtgggcattgaatgatacggtggagggggaattgtgagggagcaatgaaatcgcggtggtccaatttggggagaggctcagcaaactcgggcaagatgggtgtaccgcgtttccaatgtgaagagccgaaagcaggacagggaaggatgctgtgtgggggacagggatagggaaaggctgaggggcagaggaaactggggtgctgagagttggtagcctgcccaccactccccacccccagtcccagtcccactcgtacctgacggtggcctcacggccccagctgcctgccccacgagcagctgccacaccagcccggactgtcagcgcaggcccatccagatggaggcctcagcccagtgcccgcctgaccggtttgcctgcctgtccccgccccttccccagcgcctgcctgtcccagtgctctctgctctcgaggactgggactccgactggactcagtcttgtgtccccatccctggtaaggaacggagatgcatcccgcagcactgcctcaatctccttaaggcagccacaggcccaggcacttctgctggtgtgggggggacagggagctgggatgccagctcctccgtggcccaggtatgtgaccttgggcaggtgacttcactctccgagccatggcttcctcattgctgagtgggcacctgcctctcgtggctgtcgcgagggaggcactgggtgggagtcccctcagctcagggcctggcgcacctgacccggggctgtgctgacccatttacctggcgctgttctaaatggatgtccataggacaagggcaacagcacacacatcaaggcttgctacaccatagccccgtcttcctctccaccacccagggggccaggtgtgatgcccgcttcacagatgaggacactgaggcccagagaagtgaagtcctcggccccagggcacacagaggcagggcggggatttggaagcagtcagtggttgctactcccaggctcgccaaggctctgtctcctgccctcggggccagcactcagtgactgcctccccacagatgccctctgaggggtgagggccggggtaaggctgggcaggagatgccctgaaggcccctcggctctctggggccccggctccctgtggctgctggcgtaacggggtcaacagttgcttccctgacagacggggtgctccgatggggatgggggaggcagccccagaacagtgcccaggacaagataaagggaacccacccagccctgagttctgcccaggtgaccaaacactgctccctacggccagagccagggcccttcctgcgacctgggaccccgtctcctcccccacccttcaagccggttgctctgggaaggttcctccctggcccaccagggaggcggggctggcatctgagcgtgggcatctgcagtgggcctccgtgccaaccccccacacccccggcccgatcatgaagcgtggcccaatgtaaatgagccgtctccgcaggacgagattgccccgggctgggagcacagtggccaggaggctgctggacactagggggagcaggcgtttggggagtgggccaggcgggcagcactgcagaggcagacacaggacacagctacactcagccaggtggaataggaaggggtgacccaggcagggcctgacggggtgactggaccccactctacaggggaggttctttagcaaggggcccctttctcatcccatttggggttcacccccagccttggtgggcagctctgagcctggggcacttacccatgtcaggcagcgggcggcgaagcccaggagtccccagatgctacagatgcgagcggggtgggagggggcagcataagggccactctgcccagggacgggcagcaggagtgcgtaggggccgcgtgtgtccatgggggtgtctggcctccccctaccccatgcatccccagccctggcagccccagcccgacctggcctacactccgggcactcccagccctgctccccaggaagacgctccgttctgtgcacatcgccgggcagagggcagccccagacttgttgacttggcagaggtgccagtaaggccgcccatgccggaggccagcatccctctgccaggagcacggggagggagggagtggagggggacgtggcagggg

SEQ ID NO: 9386 - RNA, 5815 nt, Homo sapiens
  source 1..5815: mol_type = other RNA
aggagagtggattccaggtggtaagaaacaaacccaactgaaactggcttaagggaggctacagggatatattgaccccaaccacacatctacagaaacagacttaacggtgtcacgaggccccatccttctccctctgaggccagctctccctgactgctgggaaacagctcccaggaggtccaggcgtatcctaccagcttagtcagtccaggaatgggaaacagcacctctgcttgcccagccccagggaagatcatagagggctcccactgacctgcatgcacctgtgacaattgctgtggccagagaactccggtgctgcagccagacctggatgctatgcccagccttggaactaaagaactgtgaggtcagtgacccagtcccatggcctgagggtgtgtgcctttgcagagctctcaggttcctcgggggctgtcccctccaccagcctcagggccctggctcagaagccacaccctcagcctcatcccagggtatgttcagtgttggcccttgtggcccctgccggcacacacttggaactgggccaggcaccccagggcctgagcgtgtggctgaacatttgaccagtgaggaatcaggaactgcccagaggagtgacacccacccccagcccagggctctgcccagagggaaagtgggggagccctagtgtaacccctcctggctggctgtggcttgggccctgtatgtccccatctctgcccaacttccctgtcctcatcagggggctgatgcagtggcttcagtgtcagtgactaaccagtggccctggagtgactcgtaaggcaggtaccctgtggacagttatttgtctgggggaggttagtgccacccactccagctggctgaggtgccagcgaggtctaacccattacgttgagaatggagccaccctaggggtggagcagcttgctgaggtcaccgaggtcatcctcagaaatgccagcccctgccctactcacagaggggcaagctagggcatggggacaaggactgggattccctgaggcctgggcgctccatgttgcctgagtcaacctggcccatccacctgtcatctctgcagcctcacccaccacccccgcagcctctcctgccacagagatgccagatgaggaggccagcatggtgcagaggagtaagtgggcttagcaggatggggcaggccctgtggcaggacggggcaggcctggtccctggtcagatcaggatgcggagagcaactccgggctctcaacacctccatttattgcatgtataccctgacttcctcactggtccttctgtgcctgctctcatgctggcaccggcttgtggccgcactccttggaagctatgtccacggctctggctcaggttcacctgggggtgtgggcctcacagggctcattcggaccctgggttgcggccccagtccagccccctattctcccatctgggcagatggaggaacccttgcctcctgctgcccgccaagtcctccatttaaggcccacctgggctggattgccctggacggaagagcgcacaggccaccggccatagcttgcccctgtgggccaagtccccagtgtggtggccttcgccggcttgccctgaggcacggcccgacgggggcgccctggaggcgctgttggcccggtgggcagcgtggggggtatcgcgggtaggggacttgggcgggctgggcggcttgagcgcgctgacggctcggatgagacccatgcgccggcggatggagtggtccaggttgaccgtgcagcgcagcaggctctgcgcctcggccacggtgaaggggaagtcggcgcccaggaagcgctcgaagagctcggggtcgccgtccaggtcgagcacgttctgcaacgccttggtcatggtgtgcagctcgcggctgttgtcgcggaaaacgtcccagaggcgcgcgcggccctcgggcgcgcccccggtctgctgccggtcctccaggcactgcagcgcccagctcaggcggcacggccactggttggcgagcaccacccacgccaccgcctggcgcggcgtggggcccccaaagtccccctgctgctgctgctgctgcagcaggcgcacggtgatgggcacggtgttgacgatgcgccgcatggacaccacgttgtcgggcacgtactcgtagaggcagtcgcgctcgtcgtgaaggcagaagagcgcctcctggattcgccgcgccgcctcgtcgtcgatgcggccctgcccgcgctccgtccccgcctgcgcctgcaccgccagcagctgcgcgctctcgcccccggcgtcccccggcagccacggcttgcgcgtcatctcgcggtacaacaggtcgtcgcggctctgcaccgcatcgtgcaggaactgcagcttggtgcggcggcccataatgggcacagagaagggcagcgtgacagtgcggttgaggaagaggtagccgttatcggccgtgcccttcatgttgcccgcgctctctaggcacgcggccaggatgctggggtccacgaccaggatgaagatgaagggcgcgtggctgtcggacagcagcgtgttgatggcgttgagcacgcccaccacgcgctccgggtagcacgtgtccagcccggtgacctccagcaccacgcgcagcctgcgccgctggtagatctccaggaagcacaggaagtcggtgagcagctccacctccttcttcacctcgcacatgaaacccagctggctgccgaacttttcacgcgacaccagccgctcgatcttcttgcgctggcttacgaacaggtgcttgcccaccgagtacacggccatgagcagccccgagcccgacagtgtggtggccgcgccgccaaacaccttgagcaggctgccgctcgggctgccgtggcccagcgcgtggccgcccagtgacaagtagagcagccccacacccaggcccagcgccgccagcagcgccagcagccccaggcacacgcggcgccgacaatgccactcgctctggcagcagtcctgcctggtggccggcttgttgcccagcaccgagtacacgctgaagggcagtgcgccatagtggcggcggatgccctcgcacaacgtggtcaccaggccggcccacagcttgtcggtgcccgcgtactgccaggcgctaaagcggatgaaaaggaactgcacgttcctgcgccgcaggtgcacctcggtgatgatgggctgcaggaacaccaggtaccacagtagctgcgggacgccccagccgctcacggcacgcggccgccactgcacgtgctgcagctcctcgctctcgcgctgcgcggcctcctgctgcatcagcgccgtgatcttgtccagcatcatgtgcaggcggcagccgaaaggggcatagaaacccacggtcacagggaccggcacgtggcagagtgtcttggccaggcagctgcagtagacgtcatcctctgtcaggatgtcttttcggtgccccaactctgggtcccagaagtagtgcccgttggggctctgggcatccttggcgaagtggactttgtaatgtttgtgcatggcagccgggcagctgggtgctgggggcctgctcctgaggcaggagggagcacacaggcttggcgtagcctctgtgggcattgaatgatacggtggagggggaattgtgagggagcaatgaaatcgcggtggtccaatttggggagaggctcagcaaactcgggcaagatgggtgtaccgcgtttccaatgtgaagagccgaaagcaggacagggaaggatgctgtgtgggggacagggatagggaaaggctgaggggcagaggaaactggggtgctgagagttggtagcctgcccaccactccccacccccagtcccagtcccactcgtacctgacggtggcctcacggccccagctgcctgccccacgagcagctgccacaccagcccggactgtcagcgcaggcccatccagatggaggcctcagcccagtgcccgcctgaccggtttgcctgcctgtccccgccccttccccagcgcctgcctgtcccagtgctctctgctctcgaggactgggactccgactggactcagtcttgtgtccccatccctggtaaggaacggagatgcatcccgcagcactgcctcaatctccttaaggcagccacaggcccaggcacttctgctggtgtgggggggacagggagctgggatgccagctcctccgtggcccaggtatgtgaccttgggcaggtgacttcactctccgagccatggcttcctcattgctgagtgggcacctgcctctcgtggctgtcgcgagggaggcactgggtgggagtcccctcagctcagggcctggcgcacctgacccggggctgtgctgacccatttacctggcgctgttctaaatggatgtccataggacaagggcaacagcacacacatcaaggcttgctacaccatagccccgtcttcctctccaccacccagggggccaggtgtgatgcccgcttcacagatgaggacactgaggcccagagaagtgaagtcctcggccccagggcacacagaggcagggcggggatttggaagcagtcagtggttgctactcccaggctcgccaaggctctgtctcctgccctcggggccagcactcagtgactgcctccccacagatgccctctgaggggtgagggccggggtaaggctgggcaggagatgccctgaaggcccctcggctctctggggccccggctccctgtggctgctggcgtaacggggtcaacagttgcttccctgacagacggggtgctccgatggggatgggggaggcagccccagaacagtgcccaggacaagataaagggaacccacccagccctgagttctgcccaggtgaccaaacactgctccctacggccagagccagggcccttcctgcgacctgggaccccgtctcctcccccacccttcaagccggttgctctgggaaggttcctccctggcccaccagggaggcggggctggcatctgagcgtgggcatctgcagtgggcctccgtgccaaccccccacacccccggcccgatcatgaagcgtggcccaatgtaaatgagccgtctccgcaggacgagattgccccgggctgggagcacagtggccaggaggctgctggacactagggggagcaggcgtttggggagtgggccaggcgggcagcactgcagaggcagacacaggacacagctacactcagccaggtggaataggaaggggtgacccaggcagggcctgacggggtgactggaccccactctacaggggaggttctttagcaaggggcccctttctcatcccatttggggttcacccccagccttggtgggcagctctgagcctggggcacttacccatgtcaggcagcgggcggcgaagcccaggagtccccagatgctacagatgcgagcggggtgggagggggcagcataagggccactctgcccagggacgggcagcaggagtgcgtaggggccgcgtgtgtccatgggggtgtctggcctccccctaccccatgcatccccagccctggcagccccagcccgacctggcctacactccgggcactcccagccctgctccccaggaagacgctccgttctgtgcacatcgccgggcagagggcagccccagacttgttgacttggcagaggtgccagtaaggccgcccatgccggaggccagcatccctctgccaggagcacggggagggagggagtggagggggacgtggcagggg

SEQ ID NO: 9387 - RNA, 2240 nt, Homo sapiens
  source 1..2240: mol_type = other RNA
aggagagtggattccaggtggttctcacaattcccagaaatgataagagtggctcaccacgcctatactgtgtaaacaataaggttcatgctgaacacctgcttgctttctggaagtctggaattttggtacatgctaggccaagggtgcttctgtaaccagtcctcagtaagagatgtgggcactgagtctctaactcacttccctgctagataacacttcacacacattgccacaaatccttcctgtgggtatccaatgggagagcactcagacgcctgcgcctgtttcctccagtctctgccccatgtaccttttccctgtgccgccatacctggtatcctttcactgccacagctgagagtcctagtgcatcactgaacctggggtggtcctggggacctcagattcagtaggatctagcagatacatcattttgttaatgttattgagaacaagatttccagcataagataaagagttacaagacactagtataaaatcaaataaatagaaacactatcaccttacatttgaattggaaataccagtatgaactcacaactttttcatttcttaaaaaatgtttattttctatttctgtttattgaaaggcctagatgcaatcacagctcagtagcactgaaaacttctaatgtcccaactgtagcctctagatactattttctagctaaaaagaaccagagcattttagagaaatgactgattccaagactggggcaggaaatgtacaaaatgagcctggggccaggcgcagtggctcatgcctataattccagcactttgggagctcaaggcaagtggatggcttgagcccaagagtttgtgaccagcctgggcaacatggcaaaaccgtgtctctactaaaaatacaaaaattagccagccatggtggcacacctgtagtcccagctacttgggaggctgaagcaggagaattgcttgaacttgggagacagagattgcagtgagctgtgattgtgccactgcactccagcctgggcaacagacaagaccctgtctcgcacacacacaaaaaagagcctgtgacatcttattgaaccatgaagcaaggaagctatcaaagactaatgaagtatgacaaagaacaaagacatcaacttaaaggggctcccactgaacataaaaaacaaattaatggcagataagtgccctcaaaaaaaaaaaactaaaacatattaaatatattaaaaatatgttcagaatgctatgaaaaccaaagcttcattggtcatcattggaagttgctagagtctgaactcacaactttgaaaattgataaataaagggaaagaaccaagcatttttcctgcttttcattatgaagagcaattcagagtaatcatacaagtgataaggaaaaggtctttgttaaagaattccagctaacagatgcagaaggaaataatggatctaagcaacgaccatcaatggatgctaaaaccgcttaggtgaaagactgaccggatttttataatggagggatcagctgataccacctaaacccaccgatcaatccaagaatctctaaatgtgcagcagccagacaccacctgcttgttgatgccacacagtagggagtacatagcaccagctctgaggtattcgtacccaataacctgactggaatggaatcaggcctctacatggaactccgcctcgtgggacttgggaatgggtacgatgatggccagcacacagatgagctggaagatggctcccaggaagagtccgtaccgtagcaggttctccaggaaagtgggctcgggcacctccggaggtgagaagtctaggtcagaggccatggcccaagtcgcttgctgcctgacgtctcttctgactcaccactctttagaaccaactgtagtcccagctactcagaaggctgaggcaggagaattgctccagctgggaggtctaggctgcagtgagccaatgagtcgtgattgcgccaccctgagtgacggggtgagagatcacacgagtattgcttccctttcagcctggtcacttcagaaggtcatgtgcctggggcaacaggatggccacttttcacatcagctctgtctaccatgggaatggccttcaaagcttgaggctctttttcttcccagccagaatcctcagagctggcagatcttcatcctcccaggaaggatttgacttctcccgcgccgccgcgccgctcccccggaagt

SEQ ID NO: 9388 - RNA, 2052 nt, Homo sapiens
  source 1..2052: mol_type = other RNA
aggagagtggattccaggtggttctcacaattcccagaaatgataagagtggctcaccacgcctatactgtgtaaacaataaggttcatgctgaacacctgcttgctttctggaagtctggaattttggtacatgctaggccaagggtgcttctgtaaccagtcctcagtaagagatgtgggcactgagtctctaactcacttccctgctagataacacttcacacacattgccacaaatccttcctgtgggtatccaatgggagagcactcagacgcctgcgcctgtttcctccagtctctgccccatgtaccttttccctgtgccgccatacctggtatcctttcactgccacagctgagagtcctagtgcatcactgaacctggggtggtcctggggacctcagattcagtaggatctagcagatacatcattttgttaatgttattgagaacaagatttccagcataagataaagagttacaagacactagtataaaatcaaataaatagaaacactatcaccttacatttgaattggaaataccagtatgaactcacaactttttcatttcttaaaaaatgtttattttctatttctgtttattgaaaggcctagatgcaatcacagctcagtagcactgaaaacttctaatgtcccaactgtagcctctagatactattttctagctaaaaagaaccagagcattttagagaaatgactgattccaagactggggcaggaaatgtacaaaatgagcctggggccaggcgcagtggctcatgcctataattccagcactttgggagctcaaggcaagtggatggcttgagcccaagagtttgtgaccagcctgggcaacatggcaaaaccgtgtctctactaaaaatacaaaaattagccagccatggtggcacacctgtagtcccagctacttgggaggctgaagcaggagaattgcttgaacttgggagacagagattgcagtgagctgtgattgtgccactgcactccagcctgggcaacagacaagaccctgtctcgcacacacacaaaaaagagcctgtgacatcttattgaaccatgaagcaaggaagctatcaaagactaatgaagtatgacaaagaacaaagacatcaacttaaaggggctcccactgaacataaaaaacaaattaatggcagataagtgccctcaaaaaaaaaaaactaaaacatattaaatatattaaaaatatgttcagaatgctatgaaaaccaaagcttcattggtcatcattggaagttgctagagtctgaactcacaactttgaaaattgataaataaagggaaagaaccaagcatttttcctgcttttcattatgaagagcaattcagagtaatcatacaagtgataaggaaaaggtctttgttaaagaattccagctaacagatgcagaaggaaataatggatctaagcaacgaccatcaatggatgctaaaaccgcttaggtgaaagactgaccggatttttataatggagggatcagctgataccacctaaacccaccgatcaatccaagaatctctaaatgtgcagcagccagacaccacctgcttgttgatgccacacagtagggagtacatagcaccagctctgaggtattcgtacccaataacctgactggaatggaatcaggcctctacatggaactccgcctcgtgggacttgggaatgggtacgatgatggccagcacacagatgagctggaagatggctcccaggaagagtccgtaccgtagcaggttctccaggaaagtgggctcgggcacctccggaggtgagaagtctaggtcagaggccatggcccaagtcgcttgctgcctgacgtctcttctgactcaccactctttagaaccaactgtagtcccagctactcagaaggctgaggcaggagaattgctccagctgggaggtctaggctgcagtgagccaatgagtcgtgattgcgccaccctgagtgacggggtgagagatcctcccgcgccgccgcgccgctcccccggaagt

SEQ ID NO: 9389 - RNA, 387 nt, Homo sapiens
  source 1..387: mol_type = other RNA
aggagcagtgccggccaaggcgcccggggccaggagagagagatgatggcttcagcaggagtccggcgtgctccggtttcaagttccagccggtgagcccaactttggacccggcagagctgtctccagtagcttcgcctcactgggcttgggacgctgcagctcctgtccccgtttcgcttctaccaggacctccgggaggcacaaaagcaggcagctttctcctgtctgtgttggacccacgcaggactaggcccccggtccacacgcagaaagtcctagcacggaagtttggcgtccacagaccaatttgtcagcttaggaccaacgttagggctgcgtttcccgaacgacaccattgtatcaagcggccattggatcaggtct

SEQ ID NO: 9390 - RNA, 898 nt, Homo sapiens
  source 1..898: mol_type = other RNA
aggagcagtgccggccaaggcgcccggggccaggagagagagatgatggcttcagcaggagtccggcgtgctccggtttcaagttccagccggtgagcccaactttggacccggcagagctgtctccagtagcttcgcctcactgggcttgggacgctgcagctcctgtccccgtttcgcttctaccaggacctccgggaggcacaaaagcaggcagctttctcctgtctgtgttggacccacgcaggactaggcccccggtccacacgcagaaagtcctagcacggaagtttggcgtccacagaccaatttgtcagcttaggaccaacgttagggctgcgtttcccgaacgacaccattgtatcaagcggccattggatcaggtctagccacaattcgcagctgaccaatcagaaaagaaaatttggctccaggacgggaccagcgagggaccaattgaaagacaagaggcggggcccgcaggcaaaccttaaccccagagacctccgtggctgttgaaggcagagggtaatgggcgggttcgctagatcgaagcttaggtcttgaagatggggatactaaaaagcaaatccaaagccactgtgaactgcaggcggacgaccggagtcaaaatctccaggatggtttattaaaatgcgaatccccgggttcctgtgagattcaatgcgtcagggtagcgggtggagccccgaaatacgactttttaacaagctctccctacaaattctccccacacagccaggtttaagaatcactgaccgggtcgtaacagatttaaaggtggtccccacccgctccagttactccaaggctcaaggagaagcgctcatttggatcacgacccggggttcgccccacccaacaccctgcgactaag

SEQ ID NO: 9391 - RNA, 899 nt, Homo sapiens
  source 1..899: mol_type = other RNA
aggagcagtgccggccaaggcgcccggggccaggagagagagatgatggcttcagcaggagtccggcgtgctccggtttcaagttccagccggtgagcccaactttggacccggcagagctgtctccagtagcttcgcctcactgggcttgggacgctgcagctcctgtccccgtttcgcttctaccaggacctccgggaggcacaaaagcaggcagctttctcctgtctgtgttggacccacgcaggactaggcccccggtccacacgcagaaagtcctagcacggaagtttggcgtccacagaccaatttgtcagcttaggaccaacgttagggctgcgtttcccgaacgacaccattgtatcaagcggccattggatcaggtctagccacaattcgcagctgaccaatcagaaaagaaaatttggctccaggacgggaccagcgagggaccaattgaaagacaagaggcggggcccgcaggcaaaccttaaccccagagacctccgtggctgttgaaggcagagggtaatgggcgggttcgctagatcgaagcttaggtcttgaagatggggatactaaaaagcaaatccaaagccactgtgaactgcaggcggacgaccggagtcaaaatctccaggatggtttattaaaatgcgaatccccgggttcctgtgagattcaatgcgtcagggtagcgggtggagccccgaaatacgactttttaacaagctctccctacaaattctccccacacagccaggtttaagaatcactgaccgggtcgtaacagatttaaaggtggtccccacccgctccagttactccaaggctcaaggagaagcgctcatttggatcacgacccggggttcgccccacccaacaccctgcgactaaga

SEQ ID NO: 9392 - RNA, 905 nt, Homo sapiens
  source 1..905: mol_type = other RNA
aggagcagtgccggccaaggcgcccggggccaggagagagagatgatggcttcagcaggagtccggcgtgctccggtttcaagttccagccggtgagcccaactttggacccggcagagctgtctccagtagcttcgcctcactgggcttgggacgctgcagctcctgtccccgtttcgcttctaccaggacctccgggaggcacaaaagcaggcagctttctcctgtctgtgttggacccacgcaggactaggcccccggtccacacgcagaaagtcctagcacggaagtttggcgtccacagaccaatttgtcagcttaggaccaacgttagggctgcgtttcccgaacgacaccattgtatcaagcggccattggatcaggtctagccacaattcgcagctgaccaatcagaaaagaaaatttggctccaggacgggaccagcgagggaccaattgaaagacaagaggcggggcccgcaggcaaaccttaaccccagagacctccgtggctgttgaaggcagagggtaatgggcgggttcgctagatcgaagcttaggtcttgaagatggggatactaaaaagcaaatccaaagccactgtgaactgcaggcggacgaccggagtcaaaatctccaggatggtttattaaaatgcgaatccccgggttcctgtgagattcaatgcgtcagggtagcgggtggagccccgaaatacgactttttaacaagctctccctacaaattctccccacacagccaggtttaagaatcactgaccgggtcgtaacagatttaaaggtggtccccacccgctccagttactccaaggctcaaggagaagcgctcatttggatcacgacccggggttcgccccacccaacaccctgcgactaagaagcgct

SEQ ID NO: 9393 - RNA, 907 nt, Homo sapiens
  source 1..907: mol_type = other RNA
aggagcagtgccggccaaggcgcccggggccaggagagagagatgatggcttcagcaggagtccggcgtgctccggtttcaagttccagccggtgagcccaactttggacccggcagagctgtctccagtagcttcgcctcactgggcttgggacgctgcagctcctgtccccgtttcgcttctaccaggacctccgggaggcacaaaagcaggcagctttctcctgtctgtgttggacccacgcaggactaggcccccggtccacacgcagaaagtcctagcacggaagtttggcgtccacagaccaatttgtcagcttaggaccaacgttagggctgcgtttcccgaacgacaccattgtatcaagcggccattggatcaggtctagccacaattcgcagctgaccaatcagaaaagaaaatttggctccaggacgggaccagcgagggaccaattgaaagacaagaggcggggcccgcaggcaaaccttaaccccagagacctccgtggctgttgaaggcagagggtaatgggcgggttcgctagatcgaagcttaggtcttgaagatggggatactaaaaagcaaatccaaagccactgtgaactgcaggcggacgaccggagtcaaaatctccaggatggtttattaaaatgcgaatccccgggttcctgtgagattcaatgcgtcagggtagcgggtggagccccgaaatacgactttttaacaagctctccctacaaattctccccacacagccaggtttaagaatcactgaccgggtcgtaacagatttaaaggtggtccccacccgctccagttactccaaggctcaaggagaagcgctcatttggatcacgacccggggttcgccccacccaacaccctgcgactaagaagcgctta

SEQ ID NO: 9394 - RNA, 356 nt, Homo sapiens
  source 1..356: mol_type = other RNA
aggaggaggaggtcaggccgcaggcggctagcaggatacttactttgaatgaggtaatacacaatggcaaagcccccggcatagaacacaccgtggaaaaggatccttgctcccagaggcattgaccgcctgcttcctgcatacttttgccacatcatagcacaactctcttgaaaatcatcaaaggcaagttgtcagttccacatggctggggaggcctcaggaaacttccaatcatggcagaaggggaagcaggcacctctgtgagcaacagaagcaccacgctacaaagagcatgacgagttcttccaggcttgggaaagcacgggtaaatgcccgcggtcctgcgcgccagc

SEQ ID NO: 9395 - RNA, 392 nt, Homo sapiens
  source 1..392: mol_type = other RNA
aggaggaggaggtcaggccgcaggcggctagcaggatacttactttgaatgaggtaatacacaatggcaaagcccccggcatagaacacaccgtggaaaaggatccttgctcccagaggcattgaccgcctgcttcctgcatacttttgccacatcatagcacaactctcttgaaaatcatcaaaggcaagttgtcctgccgctgagttggaagacaacagctgctaacacacgaagcctcagaaagccctcgccaggactcagagattctctcgagtgactcgtgtggcaaacatcctgtgagcaacagaagcaccacgctacaaagagcatgacgagttcttccaggcttgggaaagcacgggtaaatgcccgcggtcctgcgcgccagc

SEQ ID NO: 9396 - RNA, 291 nt, Homo sapiens
  source 1..291: mol_type = other RNA
aggaggaggaggtcaggccgcaggcggctagcaggatacttactttgaatgaggtaatacacaatggcaaagcccccggcatagaacacaccgtggaaaaggatccttgctcccagaggcattgaccgcctgcttcctgcatacttttgccacatcatagcacaactctcttgaaaatcatcaaaggcaagttgtcctgtgagcaacagaagcaccacgctacaaagagcatgacgagttcttccaggcttgggaaagcacgggtaaatgcccgcggtcctgcgcgccagc

SEQ ID NO: 9397 - RNA, 511 nt, Homo sapiens
  source 1..511: mol_type = other RNA
aggaggaggaggtcaggccgcaggcggctagcaggatacttactttgaatgaggtaatacacaatggcaaagcccccggcatagaacacaccgtggaaaaggatccttgctcccagaggcattgaccgcctgcttcctgcatacttttgccacatcatagcacaactctcttgaaaatcatcaaaggcaagttgtctgtcattcactaggcatttcctcaaggtgccacatatttgacacggcttcctatctgctcaatagacagggaagcttgaggagctacaaggtccagagtgtccgtggggaaaggcaaacctgccgctgagttggaagacaacagctgctaacacacgaagcctcagaaagccctcgccaggactcagagattctctcgagtgactcgtgtggcaaacatcctgtgagcaacagaagcaccacgctacaaagagcatgacgagttcttccaggcttgggaaagcacgggtaaatgcccgcggtcctgcgcgccagc

SEQ ID NO: 9398 - RNA, 178 nt, Homo sapiens
  source 1..178: mol_type = other RNA
aggaggcagcgctctcaggacagcaccctgatcatacagaagtccacggatcagtgaggataggtgaaacttgaggctggtttcaacacaaatctgagcttgaattatacttttttcgtctctcgcggagaccgaaagattctcccagacgctgcaagcgcggctcttctcacaagac

SEQ ID NO: 9399 - RNA, 190 nt, Homo sapiens
  source 1..190: mol_type = other RNA
aggaggcagcgctctcaggacagcaccctgatcatacagaagtccacggatcagtgaggataggtgaaacttgaggctggtttcaacacaaatctgagcttgaattatacttttttcgtggaatgaagcacctctcgcggagaccgaaagattctcccagacgctgcaagcgcggctcttctcacaagac

SEQ ID NO: 9400 - RNA, 5938 nt, Homo sapiens
  source 1..5938: mol_type = other RNA
aggaggcatcttgagaaatggaaggaatgtctaactttttggatcacagtgaaacaaagtctggatcacttccagacatcaacgagcagtcgcttttacaataaaaaaaaatttttttaggtttaatttcataggtgatagatagcaatgggtctttcttgacagtgtttaatagaaagttttcctcttttcattccattacgtatgaatttttgattcattctttttaaatgacaatactaatggttgctattgagtacaagatgcagagattttgctggaggctggtaaattttctctgcaaaacagatatccccccaccccccacccccaaatttcaggtccaggtttgctatatcatcactagtccttttttaattctcactggaaattttcaaatattgtttataaactgaatgagaatgtgctatgttctctaacattcttattttacatcattctctaatatattaggaatgttgcaacaatgttatcacaatgaagtggcaacttttggcctttagactgtacctatcatcagcaatcataaaaaggccaaaataaacagtgctattccaaggtgacatctgaaactgttaaaacaagtgaaaaatcataatgacaaaacaggggttcataaagcaaaagaaaatttgccaatgcaattttaaaagtgtaagaaacttcactcatgtacctactcatgggaagaacatctaaggcaaatgaaaaattcccctccagggacataaccagctcagaaccatctgaaaaaattcatacaaaagcagaaattacccaaggcctgtgagtcctcatctcataccatgaaagccagactgtcaaaaaaagggcacatgtcactttgcaaaggaatgtattaactcctctcccagggtcaacttagtctacgtgtcttttgtataacattaatttccaccagatctactagatgttcagtcatgtcctttcaggtcctgaaggcaggctcactctctgatgcatctttttatatcatggtgggtgtgaagtgaaaagaggagacacagaaatatgcacaaacccacaattagtccatatttagaaaactttctgtgggttcaagcatttacacagagatgattttatctcatttctccattaatttcccatttgaaatgaaaaccagctaattctaaattctaaagccctgggggaaaccttccaggctttgtctatcagacagactttgtcataaaaaacacagaaaaacaaaaataaaacattacgctggaatcagcttttgagagtttgtgctttaaaaacacagtgcctaacagcaccaagcatatcatagatgctcaataaatatttgtagatttattaagagtaataacatggtgtttaaagaaccaaccaccattttgtaaaataggcaaaactacattaatttctttcacctgatttgataaagcagtgtggagcaatgaatgagagaatctgcaaattaaatatgaactctaatttgattgcagagagaaaattactgagaactttgcaaaaaacattgccacagtagccttgacactcaacagtgcaacgaagagttaatgtttccactgcaatatgaactggttcccacagctcttaggagatagagtgtaatcacttaaatgggaaatgaactctaattccacttgagaaaaggtatgttatgttcataattttatctgaaaattattaatatatttcagggagatggtcctctcattcagcatccctcaaagtaatgcaggcataagtatcaggggaccttgttatataacttcagtacagcattgtcttatacaagtgttctctcttccacatctgtagtagctgctttctaatattgtagatttttacagttgtgacacccctgggatgacagacatgagaatatggaggattaaaggttacaaaacttaaacaaaaaagggaagctcctctatgttatgtgaaaaccccttacaaaaggcagtttattgacaaataaatgctttatacattcaggtttttcccatctctcaatagtgatggtttccaaagaagaaactcagtagtgaagaatacatacttttttttttttgcattagtttgatcagttgaaaatcagaaccttcaaagcatcttgtgaatgagagaaatggaactggacctgggcaaggcatggggatggtagagatccatatgaataaatgatttagctgttgatgtggacagcaagagagttggtgggaaatgttacagcagacctgaccacgctacaaagggtctgtgaagaacacagtacaggtatcaaaacaccaaaacaaaactaaactaaaaacaagaacaaactgcaactttgccaaactgtaaacaaggtaaagcatttcacaggttcaaagttcaagggaagtaaacgtctttaaattatttttgtcagttcaaccctgatttaaaaatatggctagcaaaaacaaggaagccacagctgtcgacatcctgagcaagcatcggtctcctttgagaagctgcactcccaagcctcttctcaagctgctacacgaggaggagacacttctctcttgaattccatctcagttctctttatttccacactcttggaatacatcgattgctttccattttggtgtctacagttctggctgctatagatttagacgtggggatactggaggagggaaggcaaattctcggaggatgctccgggcaacttcgacattattctgggctatctctaaggctctcttcacctcttcaaaggcataaccctctcccatgagttttgcaatttttgcatcgacattttccaatgccgcctcaggcccatggggttttctgtggtgaatttctggtgcagtcctgcgcggtcgtggtttagggggtctggctggtgcctgtgaaccatctgaacatgaaggaagctgatcatagtcctgtgatgttctgttagttttgacattttcacctggtaaccttctagcaggaggcaaaggaacttggccacttgctagatcaacaaagggatcaccttggcagtcagagacggggcatctgaaggaagaagaaaaagatcctgtcctgaggatggccggctactggagccaggaggttttgaatgttcaatgagactatgccttgcaggaggtgggggaggtgggagagatggagggagggcatcaaaagcatcttcacctaatggagggatgagaagatcataatcagagggcgtcctgttgagtgaagaaccatgctttggattgtcccgagttggaggcctggcaggtggtaatggcacgggatcagaggctgaatcaaaaacatctccctttaaatatatgcttaagtcagggatgtttgatttcttctctgaagatggaccatgtgttccattcagcatacagtgaccattatcacaagaccgaacaggaggttttacattatgacaatgagatggttgtgaattcagggaaacagggtgggatgaaggaatcttgtattcatcatcatcttcctctactgggtctcttgttttctctgaaagagaatttgctaacggaccagtacactttatgctagggaggagggtggtaactggaggaggaggagaaagccggggaggaacatcatattcttcacttccaaggtgaccattggaaaagaccttagctccttctaaaggcaaatcatggcgtctgtgtttccgcataagcactgggtcagagcccactctactgtgccttccattgacatttgaactcgctgtgattccaggttttggagagccctcccctaggagtcgacatcccacaagctgattagtcccaaacacatcccgagggcaccatgcttcaagaggcattggcgggtctctggaaggcacgctttccacatgatggatgtgtctactcagtctattgtctggtgggattggtggaggtctttcaggtggcggtggaggaggatctcttaagggaggaggtggtgctgggagtggtttatcttgttttctcaccatgcaaggagaagactttggtgaacccgttgggctgccacagggagatctaactatgcctttctgaattagatccaggcgaggaggcacgggtggcaggcttagatgtgggatctggagtgggtcaggctgtggctttcttctctgggcaaggggagaggatcctggtgatgtgactggtgagttctgcctgtcagtgcactttcggacgtttgccaaccgattcatcatcaaggactcctcacgatcatcatcgtcgtccaagtctagcatcggcatgccaaaggggtcaatgatgctgcaacacctggagccttcatctcttggatcaaaggggtccacgattatgggctcagttccttttatttcacaacgacagaaagggcagccctgaccatccgactcctgccatgccgtaaggcaagaggtgcacatcaaatgcccacaaggctcaatcttgacatctttgtcattctctgcacaaatcttacagagctgaaaagtggagcccatttcacaatataattcatattgttcctgtgtaacttttatatggtcatgaggtgtaggttcacataatccagttaaatcaggattataactcctcccatcaggataaagataaaatccttccctgctgccatcaatcagggcttgaaataagggcttgttatgaggtatggtctgtaagatattcccatccccagtcacatagccaatggcccactgtcccaatcgagtgcaacttaaccggaaaatatagcttccgggtttggtgctatatttctgtagtcgtgctttaacttcatcatatgtgagaaatgccatgtaacctggatgtgtcacagctaagaaattccaattccgcaaaatagagccccaaggctgaaacagcctggtaaaaatatcaaattcaaaaactgaaatgtaatcattgcaagttaaatcaattgttgattttagagccattgcttccaggccagagctaatctggtggacctcatgaaggcactgtctgaatactttccatggtacgatagttttgtctccaaaaaactttctccagaattcagcagcatctgcttttgtgatacgaaagttatctccctggaattgaccattgggaaagattgctttgatttctgccagcatgtgactgaagataagggacagttttgtgagatttcgtctgtcctgtgactgttcttcatacattctctccttgccttctttaaagagtcttattgcccgttttgactttttcataaggctatcaatgtagattttaaagtactcattctcactgagttgggcaagtttctggttgtcatcatatttactcaatataagtcgtaaatgctgatatgtatcaggcaaaatatcaagtatatatggtgggctatttttcaactgaagtttgggattttggcacagtcttaccactttgtccatgagcttccaagtcttctccacggtcctgcgatctgcggcagcttgcttagggggtccaactgcatcctgaatagcatcaataatacccaaaattcgaccttttcggggatttcctcctcgaccaccagggtttctgccattcattgagtttgccatctggaattttagttctttcggcgccgtagctgtccagagacacgcgtgtgcgcgggtcccactccacacgcacgcagcccagtgtgtgtggggagccccggctgggagtgggatcgctgagaacagctcgctcccgaagaaggagcaacccagcgcgcaggcctccgagacgtggaaacgcaacaattaccgtcaagacaaatccacacccgctctcccctcccgcccgactcggggaggccgcgggacgccgcagcagcactagcaggaggaggagaccgctcgctggac

SEQ ID NO: 9401 - RNA, 5914 nt, Homo sapiens
  source 1..5914: mol_type = other RNA
aggaggcatcttgagaaatggaaggaatgtctaactttttggatcacagtgaaacaaagtctggatcacttccagacatcaacgagcagtcgcttttacaataaaaaaaaatttttttaggtttaatttcataggtgatagatagcaatgggtctttcttgacagtgtttaatagaaagttttcctcttttcattccattacgtatgaatttttgattcattctttttaaatgacaatactaatggttgctattgagtacaagatgcagagattttgctggaggctggtaaattttctctgcaaaacagatatccccccaccccccacccccaaatttcaggtccaggtttgctatatcatcactagtccttttttaattctcactggaaattttcaaatattgtttataaactgaatgagaatgtgctatgttctctaacattcttattttacatcattctctaatatattaggaatgttgcaacaatgttatcacaatgaagtggcaacttttggcctttagactgtacctatcatcagcaatcataaaaaggccaaaataaacagtgctattccaaggtgacatctgaaactgttaaaacaagtgaaaaatcataatgacaaaacaggggttcataaagcaaaagaaaatttgccaatgcaattttaaaagtgtaagaaacttcactcatgtacctactcatgggaagaacatctaaggcaaatgaaaaattcccctccagggacataaccagctcagaaccatctgaaaaaattcatacaaaagcagaaattacccaaggcctgtgagtcctcatctcataccatgaaagccagactgtcaaaaaaagggcacatgtcactttgcaaaggaatgtattaactcctctcccagggtcaacttagtctacgtgtcttttgtataacattaatttccaccagatctactagatgttcagtcatgtcctttcaggtcctgaaggcaggctcactctctgatgcatctttttatatcatggtgggtgtgaagtgaaaagaggagacacagaaatatgcacaaacccacaattagtccatatttagaaaactttctgtgggttcaagcatttacacagagatgattttatctcatttctccattaatttcccatttgaaatgaaaaccagctaattctaaattctaaagccctgggggaaaccttccaggctttgtctatcagacagactttgtcataaaaaacacagaaaaacaaaaataaaacattacgctggaatcagcttttgagagtttgtgctttaaaaacacagtgcctaacagcaccaagcatatcatagatgctcaataaatatttgtagatttattaagagtaataacatggtgtttaaagaaccaaccaccattttgtaaaataggcaaaactacattaatttctttcacctgatttgataaagcagtgtggagcaatgaatgagagaatctgcaaattaaatatgaactctaatttgattgcagagagaaaattactgagaactttgcaaaaaacattgccacagtagccttgacactcaacagtgcaacgaagagttaatgtttccactgcaatatgaactggttcccacagctcttaggagatagagtgtaatcacttaaatgggaaatgaactctaattccacttgagaaaaggtatgttatgttcataattttatctgaaaattattaatatatttcagggagatggtcctctcattcagcatccctcaaagtaatgcaggcataagtatcaggggaccttgttatataacttcagtacagcattgtcttatacaagtgttctctcttccacatctgtagtagctgctttctaatattgtagatttttacagttgtgacacccctgggatgacagacatgagaatatggaggattaaaggttacaaaacttaaacaaaaaagggaagctcctctatgttatgtgaaaaccccttacaaaaggcagtttattgacaaataaatgctttatacattcaggtttttcccatctctcaatagtgatggtttccaaagaagaaactcagtagtgaagaatacatacttttttttttttgcattagtttgatcagttgaaaatcagaaccttcaaagcatcttgtgaatgagagaaatggaactggacctgggcaaggcatggggatggtagagatccatatgaataaatgatttagctgttgatgtggacagcaagagagttggtgggaaatgttacagcagacctgaccacgctacaaagggtctgtgaagaacacagtacaggtatcaaaacaccaaaacaaaactaaactaaaaacaagaacaaactgcaactttgccaaactgtaaacaaggtaaagcatttcacaggttcaaagttcaagggaagtaaacgtctttaaattatttttgtcagttcaaccctgatttaaaaatatggctagcaaaaacaaggaagccacagctgtcgacatcctgagcaagcatcggtctcctttgagaagctgcactcccaagcctcttctcaagctgctacacgaggaggagacacttctctcttgaattccatctcagttctctttatttccacactcttggaatacatcgattgctttccattttggtgtctacagttctggctgctatagatttagacgtggggatactggaggagggaaggcaaattctcggaggatgctccgggcaacttcgacattattctgggctatctctaaggctctcttcacctcttcaaaggcataaccctctcccatgagttttgcaatttttgcatcgacattttccaatgccgcctcaggcccatggggttttctgtggtgaatttctggtgcagtcctgcgcggtcgtggtttagggggtctggctggtgcctgtgaaccatctgaacatgaaggaagctgatcatagtcctgtgatgttctgttagttttgacattttcacctggtaaccttctagcaggaggcaaaggaacttggccacttgctagatcaacaaagggatcaccttggcagtcagagacggggcatctgaaggaagaagaaaaagatcctgtcctgaggatggccggctactggagccaggaggttttgaatgttcaatgagactatgccttgcaggaggtgggggaggtgggagagatggagggagggcatcaaaagcatcttcacctaatggagggatgagaagatcataatcagagggcgtcctgttgagtgaagaaccatgctttggattgtcccgagttggaggcctggcaggtggtaatggcacgggatcagaggctgaatcaaaaacatctccctttaaatatatgcttaagtcagggatgtttgatttcttctctgaagatggaccatgtgttccattcagcatacagtgaccattatcacaagaccgaacaggaggttttacattatgacaatgagatggttgtgaattcagggaaacagggtgggatgaaggaatcttgtattcatcatcatcttcctctactgggtctcttgttttctctgaaagagaatttgctaacggaccagtacactttatgctagggaggagggtggtaactggaggaggaggagaaagccggggaggaacatcatattcttcacttccaaggtgaccattggaaaagaccttagctccttctaaaggcaaatcatggcgtctgtgtttccgcataagcactgggtcagagcccactctactgtgccttccattgacatttgaactcgctgtgattccaggttttggagagccctcccctaggagtcgacatcccacaagctgattagtcccaaacacatcccgagggcaccatgcttcaagaggcattggcgggtctctggaaggcacgctttccacatgatggatgtgtctactcagtctattgtctggtgggattggtggaggtctttcaggtggcggtggaggaggatctcttaagggaggaggtggtgctgggagtggtttatcttgttttctcaccatgcaaggagaagactttggtgaacccgttgggctgccacagggagatctaactatgcctttctgaattagatccaggcgaggaggcacgggtggcaggcttagatgtgggatctggagtgggtcaggctgtggctttcttctctgggcaaggggagaggatcctggtgatgtgactggtgagttctgcctgtcagtgcactttcggacgtttgccaaccgattcatcatcaaggactcctcacgatcatcatcgtcgtccaagtctagcatcggcatgccaaaggggtcaatgatgctgcaacacctggagccttcatctcttggatcaaaggggtccacgattatgggctcagttccttttatttcacaacgacagaaagggcagccctgaccatccgactcctgccatgccgtaaggcaagaggtgcacatcaaatgcccacaaggctcaatcttgacatctttgtcattctctgcacaaatcttacagagctgaaaagtggagcccatttcacaatataattcatattgttcctgtgtaacttttatatggtcatgaggtgtaggttcacataatccagttaaatcaggattataactcctcccatcaggataaagataaaatccttccctgctgccatcaatcagggcttgaaataagggcttgttatgaggtatggtctgtaagatattcccatccccagtcacatagccaatggcccactgtcccaatcgagtgcaacttaaccggaaaatatagcttccgggtttggtgctatatttctgtagtcgtgctttaacttcatcatatgtgagaaatgccatgtaacctggatgtgtcacagctaagaaattccaattccgcaaaatagagccccaaggctgaaacagcctggtaaaaatatcaaattcaaaaactgaaatgtaatcattgcaagttaaatcaattgttgattttagagccattgcttccaggccagagctaatctggtggacctcatgaaggcactgtctgaatactttccatggtacgatagttttgtctccaaaaaactttctccagaattcagcagcatctgcttttgtgatacgaaagttatctccctggaattgaccattgggaaagattgctttgatttctgccagcatgtgactgaagataagggacagttttgtgagatttcgtctgtcctgtgactgttcttcatacattctctccttgccttctttaaagagtcttattgcccgttttgactttttcataaggctatcaatgtagattttaaagtactcattctcactgagttgggcaagtttctggttgtcatcatatttactcaatataagtcgtaaatgctgatatgtatcaggcaaaatatcaagtatatatggtgggctatttttcaactgaagtttgggattttggcacagtcttaccactttgtccatgagcttccaagtcttctccacggtcctgcgatctgcggcagcttgcttagggggtccaactgcatcctgaatagcatcaataatacccaaaattcgaccttttcggggatttcctcctcgaccaccagggtttctgccattcattgagtttgccatctggaattttagttctttctttaaatcaacgcggtgagtcgttattcccaagaaccaaatgaaattaacacacaaatagcccatttgaaaagagaaaagagaaaaatgacaagagcggccacggaaaggaggagttcacttctctggctcctcgcctctgccctcaacccaaagctttgtttcaggacgcctgtgtcccttccctgctcaggccccttcccggcccctcgggtctgagctgcaggaggaaggtggactgggagggga

SEQ ID NO: 9402 - RNA, 5894 nt, Homo sapiens
  source 1..5894: mol_type = other RNA
aggaggcatcttgagaaatggaaggaatgtctaactttttggatcacagtgaaacaaagtctggatcacttccagacatcaacgagcagtcgcttttacaataaaaaaaaatttttttaggtttaatttcataggtgatagatagcaatgggtctttcttgacagtgtttaatagaaagttttcctcttttcattccattacgtatgaatttttgattcattctttttaaatgacaatactaatggttgctattgagtacaagatgcagagattttgctggaggctggtaaattttctctgcaaaacagatatccccccaccccccacccccaaatttcaggtccaggtttgctatatcatcactagtccttttttaattctcactggaaattttcaaatattgtttataaactgaatgagaatgtgctatgttctctaacattcttattttacatcattctctaatatattaggaatgttgcaacaatgttatcacaatgaagtggcaacttttggcctttagactgtacctatcatcagcaatcataaaaaggccaaaataaacagtgctattccaaggtgacatctgaaactgttaaaacaagtgaaaaatcataatgacaaaacaggggttcataaagcaaaagaaaatttgccaatgcaattttaaaagtgtaagaaacttcactcatgtacctactcatgggaagaacatctaaggcaaatgaaaaattcccctccagggacataaccagctcagaaccatctgaaaaaattcatacaaaagcagaaattacccaaggcctgtgagtcctcatctcataccatgaaagccagactgtcaaaaaaagggcacatgtcactttgcaaaggaatgtattaactcctctcccagggtcaacttagtctacgtgtcttttgtataacattaatttccaccagatctactagatgttcagtcatgtcctttcaggtcctgaaggcaggctcactctctgatgcatctttttatatcatggtgggtgtgaagtgaaaagaggagacacagaaatatgcacaaacccacaattagtccatatttagaaaactttctgtgggttcaagcatttacacagagatgattttatctcatttctccattaatttcccatttgaaatgaaaaccagctaattctaaattctaaagccctgggggaaaccttccaggctttgtctatcagacagactttgtcataaaaaacacagaaaaacaaaaataaaacattacgctggaatcagcttttgagagtttgtgctttaaaaacacagtgcctaacagcaccaagcatatcatagatgctcaataaatatttgtagatttattaagagtaataacatggtgtttaaagaaccaaccaccattttgtaaaataggcaaaactacattaatttctttcacctgatttgataaagcagtgtggagcaatgaatgagagaatctgcaaattaaatatgaactctaatttgattgcagagagaaaattactgagaactttgcaaaaaacattgccacagtagccttgacactcaacagtgcaacgaagagttaatgtttccactgcaatatgaactggttcccacagctcttaggagatagagtgtaatcacttaaatgggaaatgaactctaattccacttgagaaaaggtatgttatgttcataattttatctgaaaattattaatatatttcagggagatggtcctctcattcagcatccctcaaagtaatgcaggcataagtatcaggggaccttgttatataacttcagtacagcattgtcttatacaagtgttctctcttccacatctgtagtagctgctttctaatattgtagatttttacagttgtgacacccctgggatgacagacatgagaatatggaggattaaaggttacaaaacttaaacaaaaaagggaagctcctctatgttatgtgaaaaccccttacaaaaggcagtttattgacaaataaatgctttatacattcaggtttttcccatctctcaatagtgatggtttccaaagaagaaactcagtagtgaagaatacatacttttttttttttgcattagtttgatcagttgaaaatcagaaccttcaaagcatcttgtgaatgagagaaatggaactggacctgggcaaggcatggggatggtagagatccatatgaataaatgatttagctgttgatgtggacagcaagagagttggtgggaaatgttacagcagacctgaccacgctacaaagggtctgtgaagaacacagtacaggtatcaaaacaccaaaacaaaactaaactaaaaacaagaacaaactgcaactttgccaaactgtaaacaaggtaaagcatttcacaggttcaaagttcaagggaagtaaacgtctttaaattatttttgtcagttcaaccctgatttaaaaatatggctagcaaaaacaaggaagccacagctgtcgacatcctgagcaagcatcggtctcctttgagaagctgcactcccaagcctcttctcaagctgctacacgaggaggagacacttctctcttgaattccatctcagttctctttatttccacactcttggaatacatcgattgctttccattttggtgtctacagttctggctgctatagatttagacgtggggatactggaggagggaaggcaaattctcggaggatgctccgggcaacttcgacattattctgggctatctctaaggctctcttcacctcttcaaaggcataaccctctcccatgagttttgcaatttttgcatcgacattttccaatgccgcctcaggcccatggggttttctgtggtgaatttctggtgcagtcctgcgcggtcgtggtttagggggtctggctggtgcctgtgaaccatctgaacatgaaggaagctgatcatagtcctgtgatgttctgttagttttgacattttcacctggtaaccttctagcaggaggcaaaggaacttggccacttgctagatcaacaaagggatctgaaggaagaagaaaaagatcctgtcctgaggatggccggctactggagccaggaggttttgaatgttcaatgagactatgccttgcaggaggtgggggaggtgggagagatggagggagggcatcaaaagcatcttcaccctttaaatatatgcttaagtcagggatgtttgatttcttctctgaagatggaccatgtgttccattcagcatacagtgaccattatcacaagaccgaacaggaggttttacattatgacaatgagatggttgtgaattcagggaaacagggtgggatgaaggaatcttgtattcatcatcatcttcctctactgggtctcttgttttctctgaaagagaatttgctaacggaccagtacactttatgctagggaggagggtggtaactggaggaggaggagaaagccggggaggaacatcatattcttcacttccaaggtgaccattggaaaagaccttagctccttctaaaggcaaatcatggcgtctgtgtttccgcataagcactgggtcagagcccactctactgtgccttccattgacatttgaactcgctgtgattccaggttttggagagccctcccctaggagtcgacatcccacaagctgattagtcccaaacacatcccgagggcaccatgcttcaagaggcattggcgggtctctggaaggcacgctttccacatgatggatgtgtctactcagtctattgtctggtgggattggtggaggtctttcaggtggcggtggaggaggatctcttaagggaggaggtggtgctgggagtggtttatcttgttttctcaccatgcaaggagaagactttggtgaacccgttgggctgccacagggagatctaactatgcctttctgaattagatccaggcgaggaggcacgggtggcaggcttagatgtgggatctggagtgggtcaggctgtggctttcttctctgggcaaggggagaggatcctggtgatgtgactggtgagttctgcctgtcagtgcacagtcacatcctggactttgtctgagggctcacatcagatctaattatcccaggattctgacagcttgaaaactcaggcaacgatacagacttgggcaaaatctaaaacatattctttcggacgtttgccaaccgattcatcatcaaggactcctcacgatcatcatcgtcgtccaagtctagcatcggcatgccaaaggggtcaatgatgctgcaacacctggagccttcatctcttggatcaaaggggtccacgattatgggctcagttccttttatttcacaacgacagaaagggcagccctgaccatccgactcctgccatgccgtaaggcaagaggtgcacatcaaatgcccacaaggctcaatcttgacatctttgtcattctctgcacaaatcttacagagctgaaaagtggagcccatttcacaatataattcatattgttcctgtgtaacttttatatggtcatgaggtgtaggttcacataatccagttaaatcaggattataactcctcccatcaggataaagataaaatccttccctgctgccatcaatcagggcttgaaataagggcttgttatgaggtatggtctgtaagatattcccatccccagtcacatagccaatggcccactgtcccaatcgagtgcaacttaaccggaaaatatagcttccgggtttggtgctatatttctgtagtcgtgctttaacttcatcatatgtgagaaatgccatgtaacctggatgtgtcacagctaagaaattccaattccgcaaaatagagccccaaggctgaaacagcctggtaaaaatatcaaattcaaaaactgaaatgtaatcattgcaagttaaatcaattgttgattttagagccattgcttccaggccagagctaatctggtggacctcatgaaggcactgtctgaatactttccatggtacgatagttttgtctccaaaaaactttctccagaattcagcagcatctgcttttgtgatacgaaagttatctccctggaattgaccattgggaaagattgctttgatttctgccagcatgtgactgaagataagggacagttttgtgagatttcgtctgtcctgtgactgttcttcatacattctctccttgccttctttaaagagtcttattgcccgttttgactttttcataaggctatcaatgtagattttaaagtactcattctcactgagttgggcaagtttctggttgtcatcatatttactcaatataagtcgtaaatgctgatatgtatcaggcaaaatatcaagtatatatggtgggctatttttcaactgaagtttgggattttggcacagtcttaccactttgtccatgagcttccaagtcttctccacggtcctgcgatctgcggcagcttgcttagggggtccaactgcatcctgaatagcatcaataatacccaaaattcgaccttttcggggatttcctcctcgaccaccagggtttctgccattcattgagtttgccatctggaattttagttctttcggcgccgtagctgtccagagacacgcgtgtgcgcgggtcccactccacacgcacgcagcccagtgtgtgtggggagccccggctgggagtgggatcgctgagaacagctcgctcccgaagaaggagcaacccagcgcgcaggcctccgagacgtggaaacgcaacaattaccgtcaagacaaatccacacccgctctcccctcccgcccgactcggggaggccgcgggacgccgcagcagcactagcaggaggaggagaccgctcgctggac

SEQ ID NO: 9403 - RNA, 5633 nt, Homo sapiens
  source 1..5633: mol_type = other RNA
aggaggcatcttgagaaatggaaggaatgtctaactttttggatcacagtgaaacaaagtctggatcacttccagacatcaacgagcagtcgcttttacaataaaaaaaaatttttttaggtttaatttcataggtgatagatagcaatgggtctttcttgacagtgtttaatagaaagttttcctcttttcattccattacgtatgaatttttgattcattctttttaaatgacaatactaatggttgctattgagtacaagatgcagagattttgctggaggctggtaaattttctctgcaaaacagatatccccccaccccccacccccaaatttcaggtccaggtttgctatatcatcactagtccttttttaattctcactggaaattttcaaatattgtttataaactgaatgagaatgtgctatgttctctaacattcttattttacatcattctctaatatattaggaatgttgcaacaatgttatcacaatgaagtggcaacttttggcctttagactgtacctatcatcagcaatcataaaaaggccaaaataaacagtgctattccaaggtgacatctgaaactgttaaaacaagtgaaaaatcataatgacaaaacaggggttcataaagcaaaagaaaatttgccaatgcaattttaaaagtgtaagaaacttcactcatgtacctactcatgggaagaacatctaaggcaaatgaaaaattcccctccagggacataaccagctcagaaccatctgaaaaaattcatacaaaagcagaaattacccaaggcctgtgagtcctcatctcataccatgaaagccagactgtcaaaaaaagggcacatgtcactttgcaaaggaatgtattaactcctctcccagggtcaacttagtctacgtgtcttttgtataacattaatttccaccagatctactagatgttcagtcatgtcctttcaggtcctgaaggcaggctcactctctgatgcatctttttatatcatggtgggtgtgaagtgaaaagaggagacacagaaatatgcacaaacccacaattagtccatatttagaaaactttctgtgggttcaagcatttacacagagatgattttatctcatttctccattaatttcccatttgaaatgaaaaccagctaattctaaattctaaagccctgggggaaaccttccaggctttgtctatcagacagactttgtcataaaaaacacagaaaaacaaaaataaaacattacgctggaatcagcttttgagagtttgtgctttaaaaacacagtgcctaacagcaccaagcatatcatagatgctcaataaatatttgtagatttattaagagtaataacatggtgtttaaagaaccaaccaccattttgtaaaataggcaaaactacattaatttctttcacctgatttgataaagcagtgtggagcaatgaatgagagaatctgcaaattaaatatgaactctaatttgattgcagagagaaaattactgagaactttgcaaaaaacattgccacagtagccttgacactcaacagtgcaacgaagagttaatgtttccactgcaatatgaactggttcccacagctcttaggagatagagtgtaatcacttaaatgggaaatgaactctaattccacttgagaaaaggtatgttatgttcataattttatctgaaaattattaatatatttcagggagatggtcctctcattcagcatccctcaaagtaatgcaggcataagtatcaggggaccttgttatataacttcagtacagcattgtcttatacaagtgttctctcttccacatctgtagtagctgctttctaatattgtagatttttacagttgtgacacccctgggatgacagacatgagaatatggaggattaaaggttacaaaacttaaacaaaaaagggaagctcctctatgttatgtgaaaaccccttacaaaaggcagtttattgacaaataaatgctttatacattcaggtttttcccatctctcaatagtgatggtttccaaagaagaaactcagtagtgaagaatacatacttttttttttttgcattagtttgatcagttgaaaatcagaaccttcaaagcatcttgtgaatgagagaaatggaactggacctgggcaaggcatggggatggtagagatccatatgaataaatgatttagctgttgatgtggacagcaagagagttggtgggaaatgttacagcagacctgaccacgctacaaagggtctgtgaagaacacagtacaggtatcaaaacaccaaaacaaaactaaactaaaaacaagaacaaactgcaactttgccaaactgtaaacaaggtaaagcatttcacaggttcaaagttcaagggaagtaaacgtctttaaattatttttgtcagttcaaccctgatttaaaaatatggctagcaaaaacaaggaagccacagctgtcgacatcctgagcaagcatcggtctcctttgagaagctgcactcccaagcctcttctcaagctgctacacgaggaggagacacttctctcttgaattccatctcagttctctttatttccacactcttggaatacatcgattgctttccattttggtgtctacagttctggctgctatagatttagacgtggggatactggaggagggaaggcaaattctcggaggatgctccgggcaacttcgacattattctgggctatctctaaggctctcttcacctcttcaaaggcataaccctctcccatgagttttgcaatttttgcatcgacattttccaatgccgcctcaggcccatggggttttctgtggtgaatttctggtgcagtcctgcgcggtcgtggtttagggggtctggctggtgcctgtgaaccatctgaacatgaaggaagctgatcatagtcctgtgatgttctgttagttttgacattttcacctggtaaccttctagcaggaggcaaaggaacttggccacttgctagatcaacaaagggatctgaaggaagaagaaaaagatcctgtcctgaggatggccggctactggagccaggaggttttgaatgttcaatgagactatgccttgcaggaggtgggggaggtgggagagatggagggagggcatcaaaagcatcttcaccctttaaatatatgcttaagtcagggatgtttgatttcttctctgaagatggaccatgtgttccattcagcatacagtgaccattatcacaagaccgaacaggaggttttacattatgacaatgagatggttgtgaattcagggaaacagggtgggatgaaggaatcttgtattcatcatcatcttcctctactgggtctcttgttttctctgaaagagaatttgctaacggaccagtacactttatgctagggaggagggtggtaactggaggaggaggagaaagccggggaggaacatcatattcttcacttccaaggtgaccattggaaaagaccttagctccttctaaaggcaaatcatggcgtctgtgtttccgcataagcactgggtcagagcccactctactgtgccttccattgacatttgaactcgctgtgattccaggttttggagagccctcccctaggagtcgacatcccacaagctgattagtcccaaacacatcccgagggcaccatgcttcaagaggcattggcgggtctctggaaggcacgctttccacatgatggatgtgtctactcagtctattgtctggtgggattggtggaggtctttcaggtggcggtggaggaggatctcttaagggaggaggtggtgctgggagtggtttatcttgttttctcaccatgcaaggagaagactttggtgaacccgttgggctgccacagggagatctaactatgcctttctgaattagatccaggcgaggaggcacgggtggcaggcttagatgtgggatctggagtgggtcaggctgtggctttcttctctgggcaaggggagaggatcctggtgatgtgactggtgagttctgcctgtcagtgcactttcggacgtttgccaaccgattcatcatcaaggactcctcacgatcatcatcgtcgtccaagtctagcatcggcatgccaaaggggtcaatgatgctgcaacacctggagccttcatctcttggatcaaaggggtccacgattatgggctcagttccttttatttcacaacgacagaaagggcagccctgaccatccgactcctgccatgccgtaaggcaagaggtgcacatcaaatgcccacaaggctcaatcttgacatctttgtcattctctgcacaaatcttacagagctgaaaagtggagcccatttcacaatataattcatattgttcctgtgtaacttttatatggtcatgaggtgtaggttcacataatccagttaaatcaggattataactcctcccatcaggataaagataaaatccttccctgctgccatcaatcagggcttgaaataagggcttgttatgaggtatggtctgtaagatattcccatccccagtcacatagccaatggcccactgtcccaatcgagtgcaacttaaccggaaaatatagcttccgggtttggtgctatatttctgtagtcgtgctttaacttcatcatatgtgagaaatgccatgtaacctggatgtgtcacagctaagaaattccaattccgcaaaatagagccccaaggctgaaacagcctggtaaaaatatcaaattcaaaaactgaaatgtaatcattgcaagttaaatcaattgttgattttagagccattgcttccaggccagagctaatctggtggacctcatgaaggcactgtctgaatactttccatggtacgatagttctgtcctgtgactgttcttcatacattctctccttgccttctttaaagagtcttattgcccgttttgactttttcataaggctatcaatgtagattttaaagtactcattctcactgagttgggcaagtttctggttgtcatcatatttactcaatataagtcgtaaatgctgatatgtatcaggcaaaatatcaagtatatatggtgggctatttttcaactgaagtttgggattttggcacagtcttaccactttgtccatgagcttccaagtcttctccacggtcctgcgatctgcggcagcttgcttagggggtccaactgcatcctgaatagcatcaataatacccaaaattcgaccttttcggggatttcctcctcgaccaccagggtttctgccattcattgagtttgccatctggaattttagttctttcggcgccgtagctgtccagagacacgcgtgtgcgcgggtcccactccacacgcacgcagcccagtgtgtgtggggagccccggctgggagtgggatcgctgagaacagctcgctcccgaagaaggagcaacccagcgcgcaggcctccgagacgtggaaacgcaacaattaccgtcaagacaaatccacacccgctctcccctcccgcccgactcggggaggccgcgggacgccgcagcagcactagcaggaggaggagaccgctcgctggac

SEQ ID NO: 9404 - RNA, 5608 nt, Homo sapiens
  source 1..5608: mol_type = other RNA
aggaggcatcttgagaaatggaaggaatgtctaactttttggatcacagtgaaacaaagtctggatcacttccagacatcaacgagcagtcgcttttacaataaaaaaaaatttttttaggtttaatttcataggtgatagatagcaatgggtctttcttgacagtgtttaatagaaagttttcctcttttcattccattacgtatgaatttttgattcattctttttaaatgacaatactaatggttgctattgagtacaagatgcagagattttgctggaggctggtaaattttctctgcaaaacagatatccccccaccccccacccccaaatttcaggtccaggtttgctatatcatcactagtccttttttaattctcactggaaattttcaaatattgtttataaactgaatgagaatgtgctatgttctctaacattcttattttacatcattctctaatatattaggaatgttgcaacaatgttatcacaatgaagtggcaacttttggcctttagactgtacctatcatcagcaatcataaaaaggccaaaataaacagtgctattccaaggtgacatctgaaactgttaaaacaagtgaaaaatcataatgacaaaacaggggttcataaagcaaaagaaaatttgccaatgcaattttaaaagtgtaagaaacttcactcatgtacctactcatgggaagaacatctaaggcaaatgaaaaattcccctccagggacataaccagctcagaaccatctgaaaaaattcatacaaaagcagaaattacccaaggcctgtgagtcctcatctcataccatgaaagccagactgtcaaaaaaagggcacatgtcactttgcaaaggaatgtattaactcctctcccagggtcaacttagtctacgtgtcttttgtataacattaatttccaccagatctactagatgttcagtcatgtcctttcaggtcctgaaggcaggctcactctctgatgcatctttttatatcatggtgggtgtgaagtgaaaagaggagacacagaaatatgcacaaacccacaattagtccatatttagaaaactttctgtgggttcaagcatttacacagagatgattttatctcatttctccattaatttcccatttgaaatgaaaaccagctaattctaaattctaaagccctgggggaaaccttccaggctttgtctatcagacagactttgtcataaaaaacacagaaaaacaaaaataaaacattacgctggaatcagcttttgagagtttgtgctttaaaaacacagtgcctaacagcaccaagcatatcatagatgctcaataaatatttgtagatttattaagagtaataacatggtgtttaaagaaccaaccaccattttgtaaaataggcaaaactacattaatttctttcacctgatttgataaagcagtgtggagcaatgaatgagagaatctgcaaattaaatatgaactctaatttgattgcagagagaaaattactgagaactttgcaaaaaacattgccacagtagccttgacactcaacagtgcaacgaagagttaatgtttccactgcaatatgaactggttcccacagctcttaggagatagagtgtaatcacttaaatgggaaatgaactctaattccacttgagaaaaggtatgttatgttcataattttatctgaaaattattaatatatttcagggagatggtcctctcattcagcatccctcaaagtaatgcaggcataagtatcaggggaccttgttatataacttcagtacagcattgtcttatacaagtgttctctcttccacatctgtagtagctgctttctaatattgtagatttttacagttgtgacacccctgggatgacagacatgagaatatggaggattaaaggttacaaaacttaaacaaaaaagggaagctcctctatgttatgtgaaaaccccttacaaaaggcagtttattgacaaataaatgctttatacattcaggtttttcccatctctcaatagtgatggtttccaaagaagaaactcagtagtgaagaatacatacttttttttttttgcattagtttgatcagttgaaaatcagaaccttcaaagcatcttgtgaatgagagaaatggaactggacctgggcaaggcatggggatggtagagatccatatgaataaatgatttagctgttgatgtggacagcaagagagttggtgggaaatgttacagcagacctgaccacgctacaaagggtctgtgaagaacacagtacaggtatcaaaacaccaaaacaaaactaaactaaaaacaagaacaaactgcaactttgccaaactgtaaacaaggtaaagcatttcacaggttcaaagttcaagggaagtaaacgtctttaaattatttttgtcagttcaaccctgatttaaaaatatggctagcaaaaacaaggaagccacagctgtcgacatcctgagcaagcatcggtctcctttgagaagctgcactcccaagcctcttctcaagctgctacacgaggaggagacacttctctcttgaattccatctcagttctctttatttccacactcttggaatacatcgattgctttccattttggtgtctacagttctggctgctatagatttagacgtggggatactggaggagggaaggcaaattctcggaggatgctccgggcaacttcgacattattctgggctatctctaaggctctcttcacctcttcaaaggcataaccctctcccatgagttttgcaatttttgcatcgacattttccaatgccgcctcaggcccatggggttttctgtggtgaatttctggtgcagtcctgcgcggtcgtggtttagggggtctggctggtgcctgtgaaccatctgaacatgaaggaagctgatcatagtcctgtgatgttctgttagttttgacattttcacctggtaaccttctagcaggaggcaaaggaacttggccacttgctagatcaacaaagggatctgaaggaagaagaaaaagatcctgtcctgaggatggccggctactggagccaggaggttttgaatgttcaatgagactatgccttgcaggaggtgggggaggtgggagagatggagggagggcatcaaaagcatcttcaccctttaaatatatgcttaagtcagggatgtttgatttcttctctgaagatggaccatgtgttccattcagcatacagtgaccattatcacaagaccgaacaggaggttttacattatgacaatgagatggttgtgaattcagggaaacagggtgggatgaaggaatcttgtattcatcatcatcttcctctactgggtctcttgttttctctgaaagagaatttgctaacggaccagtacactttatgctagggaggagggtggtaactggaggaggaggagaaagccggggaggaacatcatattcttcacttccaaggtgaccattggaaaagaccttagctccttctaaaggcaaatcatggcgtctgtgtttccgcataagcactgggtcagagcccactctactgtgccttccattgacatttgaactcgctgtgattccaggttttggagagccctcccctaggagtcgacatcccacaagctgattagtcccaaacacatcccgagggcaccatgcttcaagaggcattggcgggtctctggaaggcacgctttccacatgatggatgtgtctactcagtctattgtctggtgggattggtggaggtctttcaggtggcggtggaggaggatctcttaagggaggaggtggtgctgggagtggtttatcttgttttctcaccatgcaaggagaagactttggtgaacccgttgggctgccacagggagatctaactatgcctttctgaattagatccaggcgaggaggcacgggtggcaggcttagatgtgggatctggagtgggtcaggctgtggctttcttctctgggcaaggggagaggatcctggtgatgtgactggtgagttctgcctgtcagtgcactttcggacgtttgccaaccgattcatcatcaaggactcctcacgatcatcatcgtcgtccaagtctagcatcggcatgccaaaggggtcaatgatgctgcaacacctggagccttcatctcttggatcaaaggggtccacgattatgggctcagttccttttatttcacaacgacagaaagggcagccctgaccatccgactcctgccatgccgtaaggcaagaggtgcacatcaaatgcccacaaggctcaatcttgacatctttgtcattctctgcacaaatcttacagagctgaaaagtggagcccatttcacaatataattcatattgttcctgtgtaacttttatatggtcatgaggtgtaggttcacataatccagttaaatcaggattataactcctcccatcaggataaagataaaatccttccctgctgccatcaatcagggcttgaaataagggcttgttatgaggtatggtctgtaagatattcccatccccagtcacatagccaatggcccactgtcccaatcgagtgcaacttaaccggaaaatatagcttccgggtttggtgctatatttctgtagtcgtgctttaacttcatcatatgtgagaaatgccatgtaacctggatgtgtcacagctaagaaattccaattccgcaaaatagagccccaaggctgaaacagcctggtaaaaatatcaaattcaaaaactgaaatgtaatcattgcaagttaaatcaattgttgattttagagccattgcttccaggccagagctaatctggtggacctcatgaaggcactgtctgaatactttccatggtacgatagttctgtcctgtgactgttcttcatacattctctccttgccttctttaaagagtcttattgcccgttttgactttttcataaggctatcaatgtagattttaaagtactcattctcactgagttgggcaagtttctggttgtcatcatatttactcaatataagtcgtaaatgctgatatgtatcaggcaaaatatcaagtatatatggtgggctatttttcaactgaagtttgggattttggcacagtcttaccactttgtccatgagcttccaagtcttctccacggtcctgcgatctgcggcagcttgcttagggggtccaactgcatcctgaatagcatcaataatacccaaaattcgaccttttcggggatttcctcctcgaccaccagggtttctgccattcattgagtttgccatctggaattttagttctttctttaaatcaacgcggtgagtcgttattcccaagaaccaaatgaaattaacacacaaatagcccatttgaaaagagaaaagagaaaaatgacaagagcggccacggaaaggaggagttcacttctctggctcctcgcctctgccctcaacccaaagctttgtttcaggacgcctgtgtcccttccctgctcaggccccttcccggcccctcgggtctgagctgcaggaggaaggtggactgggagggg

SEQ ID NO: 9405 - RNA, 5568 nt, Homo sapiens
  source 1..5568: mol_type = other RNA
aggaggcatcttgagaaatggaaggaatgtctaactttttggatcacagtgaaacaaagtctggatcacttccagacatcaacgagcagtcgcttttacaataaaaaaaaatttttttaggtttaatttcataggtgatagatagcaatgggtctttcttgacagtgtttaatagaaagttttcctcttttcattccattacgtatgaatttttgattcattctttttaaatgacaatactaatggttgctattgagtacaagatgcagagattttgctggaggctggtaaattttctctgcaaaacagatatccccccaccccccacccccaaatttcaggtccaggtttgctatatcatcactagtccttttttaattctcactggaaattttcaaatattgtttataaactgaatgagaatgtgctatgttctctaacattcttattttacatcattctctaatatattaggaatgttgcaacaatgttatcacaatgaagtggcaacttttggcctttagactgtacctatcatcagcaatcataaaaaggccaaaataaacagtgctattccaaggtgacatctgaaactgttaaaacaagtgaaaaatcataatgacaaaacaggggttcataaagcaaaagaaaatttgccaatgcaattttaaaagtgtaagaaacttcactcatgtacctactcatgggaagaacatctaaggcaaatgaaaaattcccctccagggacataaccagctcagaaccatctgaaaaaattcatacaaaagcagaaattacccaaggcctgtgagtcctcatctcataccatgaaagccagactgtcaaaaaaagggcacatgtcactttgcaaaggaatgtattaactcctctcccagggtcaacttagtctacgtgtcttttgtataacattaatttccaccagatctactagatgttcagtcatgtcctttcaggtcctgaaggcaggctcactctctgatgcatctttttatatcatggtgggtgtgaagtgaaaagaggagacacagaaatatgcacaaacccacaattagtccatatttagaaaactttctgtgggttcaagcatttacacagagatgattttatctcatttctccattaatttcccatttgaaatgaaaaccagctaattctaaattctaaagccctgggggaaaccttccaggctttgtctatcagacagactttgtcataaaaaacacagaaaaacaaaaataaaacattacgctggaatcagcttttgagagtttgtgctttaaaaacacagtgcctaacagcaccaagcatatcatagatgctcaataaatatttgtagatttattaagagtaataacatggtgtttaaagaaccaaccaccattttgtaaaataggcaaaactacattaatttctttcacctgatttgataaagcagtgtggagcaatgaatgagagaatctgcaaattaaatatgaactctaatttgattgcagagagaaaattactgagaactttgcaaaaaacattgccacagtagccttgacactcaacagtgcaacgaagagttaatgtttccactgcaatatgaactggttcccacagctcttaggagatagagtgtaatcacttaaatgggaaatgaactctaattccacttgagaaaaggtatgttatgttcataattttatctgaaaattattaatatatttcagggagatggtcctctcattcagcatccctcaaagtaatgcaggcataagtatcaggggaccttgttatataacttcagtacagcattgtcttatacaagtgttctctcttccacatctgtagtagctgctttctaatattgtagatttttacagttgtgacacccctgggatgacagacatgagaatatggaggattaaaggttacaaaacttaaacaaaaaagggaagctcctctatgttatgtgaaaaccccttacaaaaggcagtttattgacaaataaatgctttatacattcaggtttttcccatctctcaatagtgatggtttccaaagaagaaactcagtagtgaagaatacatacttttttttttttgcattagtttgatcagttgaaaatcagaaccttcaaagcatcttgtgaatgagagaaatggaactggacctgggcaaggcatggggatggtagagatccatatgaataaatgatttagctgttgatgtggacagcaagagagttggtgggaaatgttacagcagacctgaccacgctacaaagggtctgtgaagaacacagtacaggtatcaaaacaccaaaacaaaactaaactaaaaacaagaacaaactgcaactttgccaaactgtaaacaaggtaaagcatttcacaggttcaaagttcaagggaagtaaacgtctttaaattatttttgtcagttcaaccctgatttaaaaatatggctagcaaaaacaaggaagccacagctgtcgacatcctgagcaagcatcggtctcctttgagaagctgcactcccaagcctcttctcaagctgctacacgaggaggagacacttctctcttgaattccatctcagttctctttatttccacactcttggaatacatcgattgctttccattttggtgtctacagttctggctgctatagatttagacgtggggatactggaggagggaaggcaaattctcggaggatgctccgggcaacttcgacattattctgggctatctctaaggctctcttcacctcttcaaaggcataaccctctcccatgagttttgcaatttttgcatcgacattttccaatgccgcctcaggcccatggggttttctgtggtgaatttctggtgcagtcctgcgcggtcgtggtttagggggtctggctggtgcctgtgaaccatctgaacatgaaggaagctgatcatagtcctgtgatgttctgttagttttgacattttcacctggtaaccttctagcaggaggcaaaggaacttggccacttgctagatcaacaaagggatctgaaggaagaagaaaaagatcctgtcctgaggatggccggctactggagccaggaggttttgaatgttcaatgagactatgccttgcaggaggtgggggaggtgggagagatggagggagggcatcaaaagcatcttcaccctttaaatatatgcttaagtcagggatgtttgatttcttctctgaagatggaccatgtgttccattcagcatacagtgaccattatcacaagaccgaacaggaggttttacattatgacaatgagatggttgtgaattcagggaaacagggtgggatgaaggaatcttgtattcatcatcatcttcctctactgggtctcttgttttctctgaaagagaatttgctaacggaccagtacactttatgctagggaggagggtggtaactggaggaggaggagaaagccggggaggaacatcatattcttcacttccaaggtgaccattggaaaagaccttagctccttctaaaggcaaatcatggcgtctgtgtttccgcataagcactgggtcagagcccactctactgtgccttccattgacatttgaactcgctgtgattccaggttttggagagccctcccctaggagtcgacatcccacaagctgattagtcccaaacacatcccgagggcaccatgcttcaagaggcattggcgggtctctggaaggcacgctttccacatgatggatgtgtctactcagtctattgtctggtgggattggtggaggtctttcaggtggcggtggaggaggatctcttaagggaggaggtggtgctgggagtggtttatcttgttttctcaccatgcaaggagaagactttggtgaacccgttgggctgccacagggagatctaactatgcctttctgaattagatccaggcgaggaggcacgggtggcaggcttagatgtgggatctggagtgggtcaggctgtggctttcttctctgggcaaggggagaggatcctggtgatgtgactggtgagttctgcctgtcagtgcactttcggacgtttgccaaccgattcatcatcaaggactcctcacgatcatcatcgtcgtccaagtctagcatcggcatgccaaaggggtcaatgatgctgcaacacctggagccttcatctcttggatcaaaggggtccacgattatgggctcagttccttttatttcacaacgacagaaagggcagccctgaccatccgactcctgccatgccgtaaggcaagaggtgcacatcaaatgcccacaaggctcaatcttgacatctttgtcattctctgcacaaatcttacagagctgaaaagtggagcccatttcacaatataattcatattgttcctgtgtaacttttatatggtcatgaggtgtaggttcacataatccagttaaatcaggattataactcctcccatcaggataaagataaaatccttccctgctgccatcaatcagggcttgaaataagggcttgttatgaggtatggtctgtaagatattcccatccccagtcacatagccaatggcccactgtcccaatcgagtgcaacttaaccggaaaatatagcttccgggtttggtgctatatttctgtagtcgtgctttaacttcatcatatgtgagaaatgccatgtaacctggatgtgtcacagctaagaaattccaattccgcaaaatagagccccaaggctgaaacagcctggtaaaaatatcaaattcaaaaactgaaatgtaatcattgcaagttaaatcaattgttgattttagagccattgcttccaggccagagctaatctggtggacctcatgaaggcactgtctgaatactttccatggtacgatagttttgtctccaaaaaactttctccagaattcagcagcatctgcttttgtgatacgaaagttatctccctggaattgaccattgggaaagattgctttgatttctgccagcatgtgactgaagataagggacagttttgtgagatttcgtctgtcctgtgactgttcttcatacattctctccttgccttctttaaagagtcttattgcccgttttgactttttcataaggctatcaatgtagattttaaagtactcattctcactgagttgggcaagtttctggttgtcatcatatttactcaatataagtcgtaaatgctgatatgtatcaggcaaaatatcaagtatatatggtgggctatttttcaactgaagtttgggattttggcacagtcttaccactttgtccatgagcttccaagtcttctccacggtcctgcgatctgcggcagcttgcttagggggtccaactgcatcctgaatagcatcaataatacccaaaattcgaccttttcggggatttcctcctcgaccaccagggtttctgccattcattgagtttgccatctggaattttagttcaataaggggtggcaggtgggcgtgagcgtcgggaccgggagccaaagccatctggggctgaaag

SEQ ID NO: 9406 - RNA, 5604 nt, Homo sapiens
  source 1..5604: mol_type = other RNA
aggaggcatcttgagaaatggaaggaatgtctaactttttggatcacagtgaaacaaagtctggatcacttccagacatcaacgagcagtcgcttttacaataaaaaaaaatttttttaggtttaatttcataggtgatagatagcaatgggtctttcttgacagtgtttaatagaaagttttcctcttttcattccattacgtatgaatttttgattcattctttttaaatgacaatactaatggttgctattgagtacaagatgcagagattttgctggaggctggtaaattttctctgcaaaacagatatccccccaccccccacccccaaatttcaggtccaggtttgctatatcatcactagtccttttttaattctcactggaaattttcaaatattgtttataaactgaatgagaatgtgctatgttctctaacattcttattttacatcattctctaatatattaggaatgttgcaacaatgttatcacaatgaagtggcaacttttggcctttagactgtacctatcatcagcaatcataaaaaggccaaaataaacagtgctattccaaggtgacatctgaaactgttaaaacaagtgaaaaatcataatgacaaaacaggggttcataaagcaaaagaaaatttgccaatgcaattttaaaagtgtaagaaacttcactcatgtacctactcatgggaagaacatctaaggcaaatgaaaaattcccctccagggacataaccagctcagaaccatctgaaaaaattcatacaaaagcagaaattacccaaggcctgtgagtcctcatctcataccatgaaagccagactgtcaaaaaaagggcacatgtcactttgcaaaggaatgtattaactcctctcccagggtcaacttagtctacgtgtcttttgtataacattaatttccaccagatctactagatgttcagtcatgtcctttcaggtcctgaaggcaggctcactctctgatgcatctttttatatcatggtgggtgtgaagtgaaaagaggagacacagaaatatgcacaaacccacaattagtccatatttagaaaactttctgtgggttcaagcatttacacagagatgattttatctcatttctccattaatttcccatttgaaatgaaaaccagctaattctaaattctaaagccctgggggaaaccttccaggctttgtctatcagacagactttgtcataaaaaacacagaaaaacaaaaataaaacattacgctggaatcagcttttgagagtttgtgctttaaaaacacagtgcctaacagcaccaagcatatcatagatgctcaataaatatttgtagatttattaagagtaataacatggtgtttaaagaaccaaccaccattttgtaaaataggcaaaactacattaatttctttcacctgatttgataaagcagtgtggagcaatgaatgagagaatctgcaaattaaatatgaactctaatttgattgcagagagaaaattactgagaactttgcaaaaaacattgccacagtagccttgacactcaacagtgcaacgaagagttaatgtttccactgcaatatgaactggttcccacagctcttaggagatagagtgtaatcacttaaatgggaaatgaactctaattccacttgagaaaaggtatgttatgttcataattttatctgaaaattattaatatatttcagggagatggtcctctcattcagcatccctcaaagtaatgcaggcataagtatcaggggaccttgttatataacttcagtacagcattgtcttatacaagtgttctctcttccacatctgtagtagctgctttctaatattgtagatttttacagttgtgacacccctgggatgacagacatgagaatatggaggattaaaggttacaaaacttaaacaaaaaagggaagctcctctatgttatgtgaaaaccccttacaaaaggcagtttattgacaaataaatgctttatacattcaggtttttcccatctctcaatagtgatggtttccaaagaagaaactcagtagtgaagaatacatacttttttttttttgcattagtttgatcagttgaaaatcagaaccttcaaagcatcttgtgaatgagagaaatggaactggacctgggcaaggcatggggatggtagagatccatatgaataaatgatttagctgttgatgtggacagcaagagagttggtgggaaatgttacagcagacctgaccacgctacaaagggtctgtgaagaacacagtacaggtatcaaaacaccaaaacaaaactaaactaaaaacaagaacaaactgcaactttgccaaactgtaaacaaggtaaagcatttcacaggttcaaagttcaagggaagtaaacgtctttaaattatttttgtcagttcaaccctgatttaaaaatatggctagcaaaaacaaggaagccacagctgtcgacatcctgagcaagcatcggtctcctttgagaagctgcactcccaagcctcttctcaagctgctacacgaggaggagacacttctctcttgaattccatctcagttctctttatttccacactcttggaatacatcgattgctttccattttggtgtctacagttctggctgctatagatttagacgtggggatactggaggagggaaggcaaattctcggaggatgctccgggcaacttcgacattattctgggctatctctaaggctctcttcacctcttcaaaggcataaccctctcccatgagttttgcaatttttgcatcgacattttccaatgccgcctcaggcccatggggttttctgtggtgaatttctggtgcagtcctgcgcggtcgtggtttagggggtctggctggtgcctgtgaaccatctgaacatgaaggaagctgatcatagtcctgtgatgttctgttagttttgacattttcacctggtaaccttctagcaggaggcaaaggaacttggccacttgctagatcaacaaagggatctgaaggaagaagaaaaagatcctgtcctgaggatggccggctactggagccaggaggttttgaatgttcaatgagactatgccttgcaggaggtgggggaggtgggagagatggagggagggcatcaaaagcatcttcaccctttaaatatatgcttaagtcagggatgtttgatttcttctctgaagatggaccatgtgttccattcagcatacagtgaccattatcacaagaccgaacaggaggttttacattatgacaatgagatggttgtgaattcagggaaacagggtgggatgaaggaatcttgtattcatcatcatcttcctctactgggtctcttgttttctctgaaagagaatttgctaacggaccagtacactttatgctagggaggagggtggtaactggaggaggaggagaaagccggggaggaacatcatattcttcacttccaaggtgaccattggaaaagaccttagctccttctaaaggcaaatcatggcgtctgtgtttccgcataagcactgggtcagagcccactctactgtgccttccattgacatttgaactcgctgtgattccaggttttggagagccctcccctaggagtcgacatcccacaagctgattagtcccaaacacatcccgagggcaccatgcttcaagaggcattggcgggtctctggaaggcacgctttccacatgatggatgtgtctactcagtctattgtctggtgggattggtggaggtctttcaggtggcggtggaggaggatctcttaagggaggaggtggtgctgggagtggtttatcttgttttctcaccatgcaaggagaagactttggtgaacccgttgggctgccacagggagatctaactatgcctttctgaattagatccaggcgaggaggcacgggtggcaggcttagatgtgggatctggagtgggtcaggctgtggctttcttctctgggcaaggggagaggatcctggtgatgtgactggtgagttctgcctgtcagtgcactttcggacgtttgccaaccgattcatcatcaaggactcctcacgatcatcatcgtcgtccaagtctagcatcggcatgccaaaggggtcaatgatgctgcaacacctggagccttcatctcttggatcaaaggggtccacgattatgggctcagttccttttatttcacaacgacagaaagggcagccctgaccatccgactcctgccatgccgtaaggcaagaggtgcacatcaaatgcccacaaggctcaatcttgacatctttgtcattctctgcacaaatcttacagagctgaaaagtggagcccatttcacaatataattcatattgttcctgtgtaacttttatatggtcatgaggtgtaggttcacataatccagttaaatcaggattataactcctcccatcaggataaagataaaatccttccctgctgccatcaatcagggcttgaaataagggcttgttatgaggtatggtctgtaagatattcccatccccagtcacatagccaatggcccactgtcccaatcgagtgcaacttaaccggaaaatatagcttccgggtttggtgctatatttctgtagtcgtgctttaacttcatcatatgtgagaaatgccatgtaacctggatgtgtcacagctaagaaattccaattccgcaaaatagagccccaaggctgaaacagcctggtaaaaatatcaaattcaaaaactgaaatgtaatcattgcaagttaaatcaattgttgattttagagccattgcttccaggccagagctaatctggtggacctcatgaaggcactgtctgaatactttccatggtacgatagttttgtctccaaaaaactttctccagaattcagcagcatctgcttttgtgatacgaaagttatctccctggaattgaccattgggaaagattgctttgatttctgccagcatgtgactgaagataagggacagttttgtgagatttcgtctgtcctgtgactgttcttcatacattctctccttgccttctttaaagagtcttattgcccgttttgactttttcataaggctatcaatgtagattttaaagtactcattctcactgagttgggcaagtttctggttgtcatcatatttactcaatataagtcgtaaatgctgatatgtatcaggcaaaatatcaagtatatatggtgggctatttttcaactgaagtttgggattttggcacagtcttaccactttgtccatgagcttccaagtcttctccacggtcctgcgatctgcggcagcttgcttagggggtccaactgcatcctgaatagcatcaataatacccaaaattcgaccttttcggggatttcctcctcgaccaccagggtttctgccattcattgagtttgccatctggaattttagttcgtcaagacaaatccacacccgctctcccctcccgcccgactcggggaggccgcgggacgccgcagcagcactagcaggaggaggagaccgctcgctggac

SEQ ID NO: 9407 - RNA, 5780 nt, Homo sapiens
  source 1..5780: mol_type = other RNA
aggaggcatcttgagaaatggaaggaatgtctaactttttggatcacagtgaaacaaagtctggatcacttccagacatcaacgagcagtcgcttttacaataaaaaaaaatttttttaggtttaatttcataggtgatagatagcaatgggtctttcttgacagtgtttaatagaaagttttcctcttttcattccattacgtatgaatttttgattcattctttttaaatgacaatactaatggttgctattgagtacaagatgcagagattttgctggaggctggtaaattttctctgcaaaacagatatccccccaccccccacccccaaatttcaggtccaggtttgctatatcatcactagtccttttttaattctcactggaaattttcaaatattgtttataaactgaatgagaatgtgctatgttctctaacattcttattttacatcattctctaatatattaggaatgttgcaacaatgttatcacaatgaagtggcaacttttggcctttagactgtacctatcatcagcaatcataaaaaggccaaaataaacagtgctattccaaggtgacatctgaaactgttaaaacaagtgaaaaatcataatgacaaaacaggggttcataaagcaaaagaaaatttgccaatgcaattttaaaagtgtaagaaacttcactcatgtacctactcatgggaagaacatctaaggcaaatgaaaaattcccctccagggacataaccagctcagaaccatctgaaaaaattcatacaaaagcagaaattacccaaggcctgtgagtcctcatctcataccatgaaagccagactgtcaaaaaaagggcacatgtcactttgcaaaggaatgtattaactcctctcccagggtcaacttagtctacgtgtcttttgtataacattaatttccaccagatctactagatgttcagtcatgtcctttcaggtcctgaaggcaggctcactctctgatgcatctttttatatcatggtgggtgtgaagtgaaaagaggagacacagaaatatgcacaaacccacaattagtccatatttagaaaactttctgtgggttcaagcatttacacagagatgattttatctcatttctccattaatttcccatttgaaatgaaaaccagctaattctaaattctaaagccctgggggaaaccttccaggctttgtctatcagacagactttgtcataaaaaacacagaaaaacaaaaataaaacattacgctggaatcagcttttgagagtttgtgctttaaaaacacagtgcctaacagcaccaagcatatcatagatgctcaataaatatttgtagatttattaagagtaataacatggtgtttaaagaaccaaccaccattttgtaaaataggcaaaactacattaatttctttcacctgatttgataaagcagtgtggagcaatgaatgagagaatctgcaaattaaatatgaactctaatttgattgcagagagaaaattactgagaactttgcaaaaaacattgccacagtagccttgacactcaacagtgcaacgaagagttaatgtttccactgcaatatgaactggttcccacagctcttaggagatagagtgtaatcacttaaatgggaaatgaactctaattccacttgagaaaaggtatgttatgttcataattttatctgaaaattattaatatatttcagggagatggtcctctcattcagcatccctcaaagtaatgcaggcataagtatcaggggaccttgttatataacttcagtacagcattgtcttatacaagtgttctctcttccacatctgtagtagctgctttctaatattgtagatttttacagttgtgacacccctgggatgacagacatgagaatatggaggattaaaggttacaaaacttaaacaaaaaagggaagctcctctatgttatgtgaaaaccccttacaaaaggcagtttattgacaaataaatgctttatacattcaggtttttcccatctctcaatagtgatggtttccaaagaagaaactcagtagtgaagaatacatacttttttttttttgcattagtttgatcagttgaaaatcagaaccttcaaagcatcttgtgaatgagagaaatggaactggacctgggcaaggcatggggatggtagagatccatatgaataaatgatttagctgttgatgtggacagcaagagagttggtgggaaatgttacagcagacctgaccacgctacaaagggtctgtgaagaacacagtacaggtatcaaaacaccaaaacaaaactaaactaaaaacaagaacaaactgcaactttgccaaactgtaaacaaggtaaagcatttcacaggttcaaagttcaagggaagtaaacgtctttaaattatttttgtcagttcaaccctgatttaaaaatatggctagcaaaaacaaggaagccacagctgtcgacatcctgagcaagcatcggtctcctttgagaagctgcactcccaagcctcttctcaagctgctacacgaggaggagacacttctctcttgaattccatctcagttctctttatttccacactcttggaatacatcgattgctttccattttggtgtctacagttctggctgctatagatttagacgtggggatactggaggagggaaggcaaattctcggaggatgctccgggcaacttcgacattattctgggctatctctaaggctctcttcacctcttcaaaggcataaccctctcccatgagttttgcaatttttgcatcgacattttccaatgccgcctcaggcccatggggttttctgtggtgaatttctggtgcagtcctgcgcggtcgtggtttagggggtctggctggtgcctgtgaaccatctgaacatgaaggaagctgatcatagtcctgtgatgttctgttagttttgacattttcacctggtaaccttctagcaggaggcaaaggaacttggccacttgctagatcaacaaagggatctgaaggaagaagaaaaagatcctgtcctgaggatggccggctactggagccaggaggttttgaatgttcaatgagactatgccttgcaggaggtgggggaggtgggagagatggagggagggcatcaaaagcatcttcaccctttaaatatatgcttaagtcagggatgtttgatttcttctctgaagatggaccatgtgttccattcagcatacagtgaccattatcacaagaccgaacaggaggttttacattatgacaatgagatggttgtgaattcagggaaacagggtgggatgaaggaatcttgtattcatcatcatcttcctctactgggtctcttgttttctctgaaagagaatttgctaacggaccagtacactttatgctagggaggagggtggtaactggaggaggaggagaaagccggggaggaacatcatattcttcacttccaaggtgaccattggaaaagaccttagctccttctaaaggcaaatcatggcgtctgtgtttccgcataagcactgggtcagagcccactctactgtgccttccattgacatttgaactcgctgtgattccaggttttggagagccctcccctaggagtcgacatcccacaagctgattagtcccaaacacatcccgagggcaccatgcttcaagaggcattggcgggtctctggaaggcacgctttccacatgatggatgtgtctactcagtctattgtctggtgggattggtggaggtctttcaggtggcggtggaggaggatctcttaagggaggaggtggtgctgggagtggtttatcttgttttctcaccatgcaaggagaagactttggtgaacccgttgggctgccacagggagatctaactatgcctttctgaattagatccaggcgaggaggcacgggtggcaggcttagatgtgggatctggagtgggtcaggctgtggctttcttctctgggcaaggggagaggatcctggtgatgtgactggtgagttctgcctgtcagtgcactttcggacgtttgccaaccgattcatcatcaaggactcctcacgatcatcatcgtcgtccaagtctagcatcggcatgccaaaggggtcaatgatgctgcaacacctggagccttcatctcttggatcaaaggggtccacgattatgggctcagttccttttatttcacaacgacagaaagggcagccctgaccatccgactcctgccatgccgtaaggcaagaggtgcacatcaaatgcccacaaggctcaatcttgacatctttgtcattctctgcacaaatcttacagagctgaaaagtggagcccatttcacaatataattcatattgttcctgtgtaacttttatatggtcatgaggtgtaggttcacataatccagttaaatcaggattataactcctcccatcaggataaagataaaatccttccctgctgccatcaatcagggcttgaaataagggcttgttatgaggtatggtctgtaagatattcccatccccagtcacatagccaatggcccactgtcccaatcgagtgcaacttaaccggaaaatatagcttccgggtttggtgctatatttctgtagtcgtgctttaacttcatcatatgtgagaaatgccatgtaacctggatgtgtcacagctaagaaattccaattccgcaaaatagagccccaaggctgaaacagcctggtaaaaatatcaaattcaaaaactgaaatgtaatcattgcaagttaaatcaattgttgattttagagccattgcttccaggccagagctaatctggtggacctcatgaaggcactgtctgaatactttccatggtacgatagttttgtctccaaaaaactttctccagaattcagcagcatctgcttttgtgatacgaaagttatctccctggaattgaccattgggaaagattgctttgatttctgccagcatgtgactgaagataagggacagttttgtgagatttcgtctgtcctgtgactgttcttcatacattctctccttgccttctttaaagagtcttattgcccgttttgactttttcataaggctatcaatgtagattttaaagtactcattctcactgagttgggcaagtttctggttgtcatcatatttactcaatataagtcgtaaatgctgatatgtatcaggcaaaatatcaagtatatatggtgggctatttttcaactgaagtttgggattttggcacagtcttaccactttgtccatgagcttccaagtcttctccacggtcctgcgatctgcggcagcttgcttagggggtccaactgcatcctgaatagcatcaataatacccaaaattcgaccttttcggggatttcctcctcgaccaccagggtttctgccattcattgagtttgccatctggaattttagttctttcggcgccgtagctgtccagagacacgcgtgtgcgcgggtcccactccacacgcacgcagcccagtgtgtgtggggagccccggctgggagtgggatcgctgagaacagctcgctcccgaagaaggagcaacccagcgcgcaggcctccgagacgtggaaacgcaacaattaccgtcaagacaaatccacacccgctctcccctcccgcccgactcggggaggccgcgggacgccgcagcagcactagcaggaggaggagaccgctcgctggac

SEQ ID NO: 9408 - RNA, 5754 nt, Homo sapiens
  source 1..5754: mol_type = other RNA
aggaggcatcttgagaaatggaaggaatgtctaactttttggatcacagtgaaacaaagtctggatcacttccagacatcaacgagcagtcgcttttacaataaaaaaaaatttttttaggtttaatttcataggtgatagatagcaatgggtctttcttgacagtgtttaatagaaagttttcctcttttcattccattacgtatgaatttttgattcattctttttaaatgacaatactaatggttgctattgagtacaagatgcagagattttgctggaggctggtaaattttctctgcaaaacagatatccccccaccccccacccccaaatttcaggtccaggtttgctatatcatcactagtccttttttaattctcactggaaattttcaaatattgtttataaactgaatgagaatgtgctatgttctctaacattcttattttacatcattctctaatatattaggaatgttgcaacaatgttatcacaatgaagtggcaacttttggcctttagactgtacctatcatcagcaatcataaaaaggccaaaataaacagtgctattccaaggtgacatctgaaactgttaaaacaagtgaaaaatcataatgacaaaacaggggttcataaagcaaaagaaaatttgccaatgcaattttaaaagtgtaagaaacttcactcatgtacctactcatgggaagaacatctaaggcaaatgaaaaattcccctccagggacataaccagctcagaaccatctgaaaaaattcatacaaaagcagaaattacccaaggcctgtgagtcctcatctcataccatgaaagccagactgtcaaaaaaagggcacatgtcactttgcaaaggaatgtattaactcctctcccagggtcaacttagtctacgtgtcttttgtataacattaatttccaccagatctactagatgttcagtcatgtcctttcaggtcctgaaggcaggctcactctctgatgcatctttttatatcatggtgggtgtgaagtgaaaagaggagacacagaaatatgcacaaacccacaattagtccatatttagaaaactttctgtgggttcaagcatttacacagagatgattttatctcatttctccattaatttcccatttgaaatgaaaaccagctaattctaaattctaaagccctgggggaaaccttccaggctttgtctatcagacagactttgtcataaaaaacacagaaaaacaaaaataaaacattacgctggaatcagcttttgagagtttgtgctttaaaaacacagtgcctaacagcaccaagcatatcatagatgctcaataaatatttgtagatttattaagagtaataacatggtgtttaaagaaccaaccaccattttgtaaaataggcaaaactacattaatttctttcacctgatttgataaagcagtgtggagcaatgaatgagagaatctgcaaattaaatatgaactctaatttgattgcagagagaaaattactgagaactttgcaaaaaacattgccacagtagccttgacactcaacagtgcaacgaagagttaatgtttccactgcaatatgaactggttcccacagctcttaggagatagagtgtaatcacttaaatgggaaatgaactctaattccacttgagaaaaggtatgttatgttcataattttatctgaaaattattaatatatttcagggagatggtcctctcattcagcatccctcaaagtaatgcaggcataagtatcaggggaccttgttatataacttcagtacagcattgtcttatacaagtgttctctcttccacatctgtagtagctgctttctaatattgtagatttttacagttgtgacacccctgggatgacagacatgagaatatggaggattaaaggttacaaaacttaaacaaaaaagggaagctcctctatgttatgtgaaaaccccttacaaaaggcagtttattgacaaataaatgctttatacattcaggtttttcccatctctcaatagtgatggtttccaaagaagaaactcagtagtgaagaatacatacttttttttttttgcattagtttgatcagttgaaaatcagaaccttcaaagcatcttgtgaatgagagaaatggaactggacctgggcaaggcatggggatggtagagatccatatgaataaatgatttagctgttgatgtggacagcaagagagttggtgggaaatgttacagcagacctgaccacgctacaaagggtctgtgaagaacacagtacaggtatcaaaacaccaaaacaaaactaaactaaaaacaagaacaaactgcaactttgccaaactgtaaacaaggtaaagcatttcacaggttcaaagttcaagggaagtaaacgtctttaaattatttttgtcagttcaaccctgatttaaaaatatggctagcaaaaacaaggaagccacagctgtcgacatcctgagcaagcatcggtctcctttgagaagctgcactcccaagcctcttctcaagctgctacacgaggaggagacacttctctcttgaattccatctcagttctctttatttccacactcttggaatacatcgattgctttccattttggtgtctacagttctggctgctatagatttagacgtggggatactggaggagggaaggcaaattctcggaggatgctccgggcaacttcgacattattctgggctatctctaaggctctcttcacctcttcaaaggcataaccctctcccatgagttttgcaatttttgcatcgacattttccaatgccgcctcaggcccatggggttttctgtggtgaatttctggtgcagtcctgcgcggtcgtggtttagggggtctggctggtgcctgtgaaccatctgaacatgaaggaagctgatcatagtcctgtgatgttctgttagttttgacattttcacctggtaaccttctagcaggaggcaaaggaacttggccacttgctagatcaacaaagggatctgaaggaagaagaaaaagatcctgtcctgaggatggccggctactggagccaggaggttttgaatgttcaatgagactatgccttgcaggaggtgggggaggtgggagagatggagggagggcatcaaaagcatcttcaccctttaaatatatgcttaagtcagggatgtttgatttcttctctgaagatggaccatgtgttccattcagcatacagtgaccattatcacaagaccgaacaggaggttttacattatgacaatgagatggttgtgaattcagggaaacagggtgggatgaaggaatcttgtattcatcatcatcttcctctactgggtctcttgttttctctgaaagagaatttgctaacggaccagtacactttatgctagggaggagggtggtaactggaggaggaggagaaagccggggaggaacatcatattcttcacttccaaggtgaccattggaaaagaccttagctccttctaaaggcaaatcatggcgtctgtgtttccgcataagcactgggtcagagcccactctactgtgccttccattgacatttgaactcgctgtgattccaggttttggagagccctcccctaggagtcgacatcccacaagctgattagtcccaaacacatcccgagggcaccatgcttcaagaggcattggcgggtctctggaaggcacgctttccacatgatggatgtgtctactcagtctattgtctggtgggattggtggaggtctttcaggtggcggtggaggaggatctcttaagggaggaggtggtgctgggagtggtttatcttgttttctcaccatgcaaggagaagactttggtgaacccgttgggctgccacagggagatctaactatgcctttctgaattagatccaggcgaggaggcacgggtggcaggcttagatgtgggatctggagtgggtcaggctgtggctttcttctctgggcaaggggagaggatcctggtgatgtgactggtgagttctgcctgtcagtgcactttcggacgtttgccaaccgattcatcatcaaggactcctcacgatcatcatcgtcgtccaagtctagcatcggcatgccaaaggggtcaatgatgctgcaacacctggagccttcatctcttggatcaaaggggtccacgattatgggctcagttccttttatttcacaacgacagaaagggcagccctgaccatccgactcctgccatgccgtaaggcaagaggtgcacatcaaatgcccacaaggctcaatcttgacatctttgtcattctctgcacaaatcttacagagctgaaaagtggagcccatttcacaatataattcatattgttcctgtgtaacttttatatggtcatgaggtgtaggttcacataatccagttaaatcaggattataactcctcccatcaggataaagataaaatccttccctgctgccatcaatcagggcttgaaataagggcttgttatgaggtatggtctgtaagatattcccatccccagtcacatagccaatggcccactgtcccaatcgagtgcaacttaaccggaaaatatagcttccgggtttggtgctatatttctgtagtcgtgctttaacttcatcatatgtgagaaatgccatgtaacctggatgtgtcacagctaagaaattccaattccgcaaaatagagccccaaggctgaaacagcctggtaaaaatatcaaattcaaaaactgaaatgtaatcattgcaagttaaatcaattgttgattttagagccattgcttccaggccagagctaatctggtggacctcatgaaggcactgtctgaatactttccatggtacgatagttttgtctccaaaaaactttctccagaattcagcagcatctgcttttgtgatacgaaagttatctccctggaattgaccattgggaaagattgctttgatttctgccagcatgtgactgaagataagggacagttttgtgagatttcgtctgtcctgtgactgttcttcatacattctctccttgccttctttaaagagtcttattgcccgttttgactttttcataaggctatcaatgtagattttaaagtactcattctcactgagttgggcaagtttctggttgtcatcatatttactcaatataagtcgtaaatgctgatatgtatcaggcaaaatatcaagtatatatggtgggctatttttcaactgaagtttgggattttggcacagtcttaccactttgtccatgagcttccaagtcttctccacggtcctgcgatctgcggcagcttgcttagggggtccaactgcatcctgaatagcatcaataatacccaaaattcgaccttttcggggatttcctcctcgaccaccagggtttctgccattcattgagtttgccatctggaattttagttctttctttaaatcaacgcggtgagtcgttattcccaagaaccaaatgaaattaacacacaaatagcccatttgaaaagagaaaagagaaaaatgacaagagcggccacggaaaggaggagttcacttctctggctcctcgcctctgccctcaacccaaagctttgtttcaggacgcctgtgtcccttccctgctcaggccccttcccggcccctcgggtctgagctgcaggaggaaggtggactgggaggg

SEQ ID NO: 9409 - RNA, 5748 nt, Homo sapiens
  source 1..5748: mol_type = other RNA
aggaggcatcttgagaaatggaaggaatgtctaactttttggatcacagtgaaacaaagtctggatcacttccagacatcaacgagcagtcgcttttacaataaaaaaaaatttttttaggtttaatttcataggtgatagatagcaatgggtctttcttgacagtgtttaatagaaagttttcctcttttcattccattacgtatgaatttttgattcattctttttaaatgacaatactaatggttgctattgagtacaagatgcagagattttgctggaggctggtaaattttctctgcaaaacagatatccccccaccccccacccccaaatttcaggtccaggtttgctatatcatcactagtccttttttaattctcactggaaattttcaaatattgtttataaactgaatgagaatgtgctatgttctctaacattcttattttacatcattctctaatatattaggaatgttgcaacaatgttatcacaatgaagtggcaacttttggcctttagactgtacctatcatcagcaatcataaaaaggccaaaataaacagtgctattccaaggtgacatctgaaactgttaaaacaagtgaaaaatcataatgacaaaacaggggttcataaagcaaaagaaaatttgccaatgcaattttaaaagtgtaagaaacttcactcatgtacctactcatgggaagaacatctaaggcaaatgaaaaattcccctccagggacataaccagctcagaaccatctgaaaaaattcatacaaaagcagaaattacccaaggcctgtgagtcctcatctcataccatgaaagccagactgtcaaaaaaagggcacatgtcactttgcaaaggaatgtattaactcctctcccagggtcaacttagtctacgtgtcttttgtataacattaatttccaccagatctactagatgttcagtcatgtcctttcaggtcctgaaggcaggctcactctctgatgcatctttttatatcatggtgggtgtgaagtgaaaagaggagacacagaaatatgcacaaacccacaattagtccatatttagaaaactttctgtgggttcaagcatttacacagagatgattttatctcatttctccattaatttcccatttgaaatgaaaaccagctaattctaaattctaaagccctgggggaaaccttccaggctttgtctatcagacagactttgtcataaaaaacacagaaaaacaaaaataaaacattacgctggaatcagcttttgagagtttgtgctttaaaaacacagtgcctaacagcaccaagcatatcatagatgctcaataaatatttgtagatttattaagagtaataacatggtgtttaaagaaccaaccaccattttgtaaaataggcaaaactacattaatttctttcacctgatttgataaagcagtgtggagcaatgaatgagagaatctgcaaattaaatatgaactctaatttgattgcagagagaaaattactgagaactttgcaaaaaacattgccacagtagccttgacactcaacagtgcaacgaagagttaatgtttccactgcaatatgaactggttcccacagctcttaggagatagagtgtaatcacttaaatgggaaatgaactctaattccacttgagaaaaggtatgttatgttcataattttatctgaaaattattaatatatttcagggagatggtcctctcattcagcatccctcaaagtaatgcaggcataagtatcaggggaccttgttatataacttcagtacagcattgtcttatacaagtgttctctcttccacatctgtagtagctgctttctaatattgtagatttttacagttgtgacacccctgggatgacagacatgagaatatggaggattaaaggttacaaaacttaaacaaaaaagggaagctcctctatgttatgtgaaaaccccttacaaaaggcagtttattgacaaataaatgctttatacattcaggtttttcccatctctcaatagtgatggtttccaaagaagaaactcagtagtgaagaatacatacttttttttttttgcattagtttgatcagttgaaaatcagaaccttcaaagcatcttgtgaatgagagaaatggaactggacctgggcaaggcatggggatggtagagatccatatgaataaatgatttagctgttgatgtggacagcaagagagttggtgggaaatgttacagcagacctgaccacgctacaaagggtctgtgaagaacacagtacaggtatcaaaacaccaaaacaaaactaaactaaaaacaagaacaaactgcaactttgccaaactgtaaacaaggtaaagcatttcacaggttcaaagttcaagggaagtaaacgtctttaaattatttttgtcagttcaaccctgatttaaaaatatggctagcaaaaacaaggaagccacagctgtcgacatcctgagcaagcatcggtctcctttgagaagctgcactcccaagcctcttctcaagctgctacacgaggaggagacacttctctcttgaattccatctcagttctctttatttccacactcttggaatacatcgattgctttccattttggtgtctacagttctggctgctatagatttagacgtggggatactggaggagggaaggcaaattctcggaggatgctccgggcaacttcgacattattctgggctatctctaaggctctcttcacctcttcaaaggcataaccctctcccatgagttttgcaatttttgcatcgacattttccaatgccgcctcaggcccatggggttttctgtggtgaatttctggtgcagtcctgcgcggtcgtggtttagggggtctggctggtgcctgtgaaccatctgaacatgaaggaagctgatcatagtcctgtgatgttctgttagttttgacattttcacctggtaaccttctagcaggaggcaaaggaacttggccacttgctagatcaacaaagggatctgaaggaagaagaaaaagatcctgtcctgaggatggccggctactggagccaggaggttttgaatgttcaatgagactatgccttgcaggaggtgggggaggtgggagagatggagggagggcatcaaaagcatcttcaccctttaaatatatgcttaagtcagggatgtttgatttcttctctgaagatggaccatgtgttccattcagcatacagtgaccattatcacaagaccgaacaggaggttttacattatgacaatgagatggttgtgaattcagggaaacagggtgggatgaaggaatcttgtattcatcatcatcttcctctactgggtctcttgttttctctgaaagagaatttgctaacggaccagtacactttatgctagggaggagggtggtaactggaggaggaggagaaagccggggaggaacatcatattcttcacttccaaggtgaccattggaaaagaccttagctccttctaaaggcaaatcatggcgtctgtgtttccgcataagcactgggtcagagcccactctactgtgccttccattgacatttgaactcgctgtgattccaggttttggagagccctcccctaggagtcgacatcccacaagctgattagtcccaaacacatcccgagggcaccatgcttcaagaggcattggcgggtctctggaaggcacgctttccacatgatggatgtgtctactcagtctattgtctggtgggattggtggaggtctttcaggtggcggtggaggaggatctcttaagggaggaggtggtgctgggagtggtttatcttgttttctcaccatgcaaggagaagactttggtgaacccgttgggctgccacagggagatctaactatgcctttctgaattagatccaggcgaggaggcacgggtggcaggcttagatgtgggatctggagtgggtcaggctgtggctttcttctctgggcaaggggagaggatcctggtgatgtgactggtgagttctgcctgtcagtgcactttcggacgtttgccaaccgattcatcatcaaggactcctcacgatcatcatcgtcgtccaagtctagcatcggcatgccaaaggggtcaatgatgctgcaacacctggagccttcatctcttggatcaaaggggtccacgattatgggctcagttccttttatttcacaacgacagaaagggcagccctgaccatccgactcctgccatgccgtaaggcaagaggtgcacatcaaatgcccacaaggctcaatcttgacatctttgtcattctctgcacaaatcttacagagctgaaaagtggagcccatttcacaatataattcatattgttcctgtgtaacttttatatggtcatgaggtgtaggttcacataatccagttaaatcaggattataactcctcccatcaggataaagataaaatccttccctgctgccatcaatcagggcttgaaataagggcttgttatgaggtatggtctgtaagatattcccatccccagtcacatagccaatggcccactgtcccaatcgagtgcaacttaaccggaaaatatagcttccgggtttggtgctatatttctgtagtcgtgctttaacttcatcatatgtgagaaatgccatgtaacctggatgtgtcacagctaagaaattccaattccgcaaaatagagccccaaggttcctagaatgagcagttaggtttaatgtaggaagattacttttactctcttccttgacaaggtgaagaagcaaagctcttactatttagaatgtctttgtatcatgttaaataaataagatattctgtaaaattatcagaaacctgaaacagcctggtaaaaatatcaaattcaaaaactgaaatgtaatcattgcaagttaaatcaattgttgattttagagccattgcttccaggccagagctaatctggtggacctcatgaaggcactgtctgaatactttccatggtacgatagttttgtctccaaaaaactttctccagaattcagcagcatctgcttttgtgatacgaaagttatctccctggaattgaccattgggaaagattgctttgatttctgccagcatgtgactgaagataagggacagttttgtgagatttcgtctgtcctgtgactgttcttcatacattctctccttgccttctttaaagagtcttattgcccgttttgactttttcataaggctatcaatgtagattttaaagtactcattctcactgagttgggcaagtttctggttgtcatcatatttactcaatataagtcgtaaatgctgatatgtatcaggcaaaatatcaagtatatatggtgggctatttttcaactgaagtttgggattttggcacagtcttaccactttgtccatgagcttccaagtcttctccacggtcctgcgatctgcggcagcttgcttagggggtccaactgcatcctgaatagcatcaataatacccaaaattcgaccttttcggggatttcctcctcgaccaccagggtttctgccattcattgagtttgccatctggaattttagttcgtcaagacaaatccacacccgctctcccctcccgcccgactcggggaggccgcgggacgccgcagcagcactagcaggaggaggagaccgctcgctggac

SEQ ID NO: 9410 - RNA, 5912 nt, Homo sapiens
  source 1..5912: mol_type = other RNA
aggaggcatcttgagaaatggaaggaatgtctaactttttggatcacagtgaaacaaagtctggatcacttccagacatcaacgagcagtcgcttttacaataaaaaaaaatttttttaggtttaatttcataggtgatagatagcaatgggtctttcttgacagtgtttaatagaaagttttcctcttttcattccattacgtatgaatttttgattcattctttttaaatgacaatactaatggttgctattgagtacaagatgcagagattttgctggaggctggtaaattttctctgcaaaacagatatccccccaccccccacccccaaatttcaggtccaggtttgctatatcatcactagtccttttttaattctcactggaaattttcaaatattgtttataaactgaatgagaatgtgctatgttctctaacattcttattttacatcattctctaatatattaggaatgttgcaacaatgttatcacaatgaagtggcaacttttggcctttagactgtacctatcatcagcaatcataaaaaggccaaaataaacagtgctattccaaggtgacatctgaaactgttaaaacaagtgaaaaatcataatgacaaaacaggggttcataaagcaaaagaaaatttgccaatgcaattttaaaagtgtaagaaacttcactcatgtacctactcatgggaagaacatctaaggcaaatgaaaaattcccctccagggacataaccagctcagaaccatctgaaaaaattcatacaaaagcagaaattacccaaggcctgtgagtcctcatctcataccatgaaagccagactgtcaaaaaaagggcacatgtcactttgcaaaggaatgtattaactcctctcccagggtcaacttagtctacgtgtcttttgtataacattaatttccaccagatctactagatgttcagtcatgtcctttcaggtcctgaaggcaggctcactctctgatgcatctttttatatcatggtgggtgtgaagtgaaaagaggagacacagaaatatgcacaaacccacaattagtccatatttagaaaactttctgtgggttcaagcatttacacagagatgattttatctcatttctccattaatttcccatttgaaatgaaaaccagctaattctaaattctaaagccctgggggaaaccttccaggctttgtctatcagacagactttgtcataaaaaacacagaaaaacaaaaataaaacattacgctggaatcagcttttgagagtttgtgctttaaaaacacagtgcctaacagcaccaagcatatcatagatgctcaataaatatttgtagatttattaagagtaataacatggtgtttaaagaaccaaccaccattttgtaaaataggcaaaactacattaatttctttcacctgatttgataaagcagtgtggagcaatgaatgagagaatctgcaaattaaatatgaactctaatttgattgcagagagaaaattactgagaactttgcaaaaaacattgccacagtagccttgacactcaacagtgcaacgaagagttaatgtttccactgcaatatgaactggttcccacagctcttaggagatagagtgtaatcacttaaatgggaaatgaactctaattccacttgagaaaaggtatgttatgttcataattttatctgaaaattattaatatatttcagggagatggtcctctcattcagcatccctcaaagtaatgcaggcataagtatcaggggaccttgttatataacttcagtacagcattgtcttatacaagtgttctctcttccacatctgtagtagctgctttctaatattgtagatttttacagttgtgacacccctgggatgacagacatgagaatatggaggattaaaggttacaaaacttaaacaaaaaagggaagctcctctatgttatgtgaaaaccccttacaaaaggcagtttattgacaaataaatgctttatacattcaggtttttcccatctctcaatagtgatggtttccaaagaagaaactcagtagtgaagaatacatacttttttttttttgcattagtttgatcagttgaaaatcagaaccttcaaagcatcttgtgaatgagagaaatggaactggacctgggcaaggcatggggatggtagagatccatatgaataaatgatttagctgttgatgtggacagcaagagagttggtgggaaatgttacagcagacctgaccacgctacaaagggtctgtgaagaacacagtacaggtatcaaaacaccaaaacaaaactaaactaaaaacaagaacaaactgcaactttgccaaactgtaaacaaggtaaagcatttcacaggttcaaagttcaagggaagtaaacgtctttaaattatttttgtcagttcaaccctgatttaaaaatatggctagcaaaaacaaggaagccacagctgtcgacatcctgagcaagcatcggtctcctttgagaagctgcactcccaagcctcttctcaagctgctacacgaggaggagacacttctctcttgaattccatctcagttctctttatttccacactcttggaatacatcgattgctttccattttggtgtctacagttctggctgctatagatttagacgtggggatactggaggagggaaggcaaattctcggaggatgctccgggcaacttcgacattattctgggctatctctaaggctctcttcacctcttcaaaggcataaccctctcccatgagttttgcaatttttgcatcgacattttccaatgccgcctcaggcccatggggttttctgtggtgaatttctggtgcagtcctgcgcggtcgtggtttagggggtctggctggtgcctgtgaaccatctgaacatgaaggaagctgatcatagtcctgtgatgttctgttagttttgacattttcacctggtaaccttctagcaggaggcaaaggaacttggccacttgctagatcaacaaagggatctgaaggaagaagaaaaagatcctgtcctgaggatggccggctactggagccaggaggttttgaatgttcaatgagactatgccttgcaggaggtgggggaggtgggagagatggagggagggcatcaaaagcatcttcaccctttaaatatatgcttaagtcagggatgtttgatttcttctctgaagatggaccatgtgttccattcagcatacagtgaccattatcacaagaccgaacaggaggttttacattatgacaatgagatggttgtgaattcagggaaacagggtgggatgaaggaatcttgtattcatcatcatcttcctctactgggtctcttgttttctctgaaagagaatttgctaacggaccagtacactttatgctagggaggagggtggtaactggaggaggaggagaaagccggggaggaacatcatattcttcacttccaaggtgaccattggaaaagaccttagctccttctaaaggcaaatcatggcgtctgtgtttccgcataagcactgggtcagagcccactctactgtgccttccattgacatttgaactcgctgtgattccaggttttggagagccctcccctaggagtcgacatcccacaagctgattagtcccaaacacatcccgagggcaccatgcttcaagaggcattggcgggtctctggaaggcacgctttccacatgatggatgtgtctactcagtctattgtctggtgggattggtggaggtctttcaggtggcggtggaggaggatctcttaagggaggaggtggtgctgggagtggtttatcttgttttctcaccatgcaaggagaagactttggtgaacccgttgggctgccacagggagatctaactatgcctttctgaattagatccaggcgaggaggcacgggtggcaggcttagatgtgggatctggagtgggtcaggctgtggctttcttctctgggcaaggggagaggatcctggtgatgtgactggtgagttctgcctgtcagtgcactttcggacgtttgccaaccgattcatcatcaaggactcctcacgatcatcatcgtcgtccaagtctagcatcggcatgccaaaggggtcaatgatgctgcaacacctggagccttcatctcttggatcaaaggggtccacgattatgggctcagttccttttatttcacaacgacagaaagggcagccctgaccatccgactccttgctatatttcatgtagctatgaggttgccacaaatctttttttaaacatagcaattataactggaaaaattatatgtatataaatgcactgagaataggttggatccataccaagaattttcaaagcacagtatctcccacagaaactcaataacttctggctgccatgccgtaaggcaagaggtgcacatcaaatgcccacaaggctcaatcttgacatctttgtcattctctgcacaaatcttacagagctgaaaagtggagcccatttcacaatataattcatattgttcctgtgtaacttttatatggtcatgaggtgtaggttcacataatccagttaaatcaggattataactcctcccatcaggataaagataaaatccttccctgctgccatcaatcagggcttgaaataagggcttgttatgaggtatggtctgtaagatattcccatccccagtcacatagccaatggcccactgtcccaatcgagtgcaacttaaccggaaaatatagcttccgggtttggtgctatatttctgtagtcgtgctttaacttcatcatatgtgagaaatgccatgtaacctggatgtgtcacagctaagaaattccaattccgcaaaatagagccccaaggttcctagaatgagcagttaggtttaatgtaggaagattacttttactctcttccttgacaaggtgaagaagcaaagctcttactatttagaatgtctttgtatcatgttaaataaataagatattctgtaaaattatcagaaacctgaaacagcctggtaaaaatatcaaattcaaaaactgaaatgtaatcattgcaagttaaatcaattgttgattttagagccattgcttccaggccagagctaatctggtggacctcatgaaggcactgtctgaatactttccatggtacgatagttttgtctccaaaaaactttctccagaattcagcagcatctgcttttgtgatacgaaagttatctccctggaattgaccattgggaaagattgctttgatttctgccagcatgtgactgaagataagggacagttttgtgagatttcgtctgtcctgtgactgttcttcatacattctctccttgccttctttaaagagtcttattgcccgttttgactttttcataaggctatcaatgtagattttaaagtactcattctcactgagttgggcaagtttctggttgtcatcatatttactcaatataagtcgtaaatgctgatatgtatcaggcaaaatatcaagtatatatggtgggctatttttcaactgaagtttgggattttggcacagtcttaccactttgtccatgagcttccaagtcttctccacggtcctgcgatctgcggcagcttgcttagggggtccaactgcatcctgaatagcatcaataatacccaaaattcgaccttttcggggatttcctcctcgaccaccagggtttctgccattcattgagtttgccatctggaattttagttcgtcaagacaaatccacacccgctctcccctcccgcccgactcggggaggccgcgggacgccgcagcagcactagcaggaggaggagaccgctcgctggac

SEQ ID NO: 9411 - RNA, 5457 nt, Homo sapiens
  source 1..5457: mol_type = other RNA
aggaggcatcttgagaaatggaaggaatgtctaactttttggatcacagtgaaacaaagtctggatcacttccagacatcaacgagcagtcgcttttacaataaaaaaaaatttttttaggtttaatttcataggtgatagatagcaatgggtctttcttgacagtgtttaatagaaagttttcctcttttcattccattacgtatgaatttttgattcattctttttaaatgacaatactaatggttgctattgagtacaagatgcagagattttgctggaggctggtaaattttctctgcaaaacagatatccccccaccccccacccccaaatttcaggtccaggtttgctatatcatcactagtccttttttaattctcactggaaattttcaaatattgtttataaactgaatgagaatgtgctatgttctctaacattcttattttacatcattctctaatatattaggaatgttgcaacaatgttatcacaatgaagtggcaacttttggcctttagactgtacctatcatcagcaatcataaaaaggccaaaataaacagtgctattccaaggtgacatctgaaactgttaaaacaagtgaaaaatcataatgacaaaacaggggttcataaagcaaaagaaaatttgccaatgcaattttaaaagtgtaagaaacttcactcatgtacctactcatgggaagaacatctaaggcaaatgaaaaattcccctccagggacataaccagctcagaaccatctgaaaaaattcatacaaaagcagaaattacccaaggcctgtgagtcctcatctcataccatgaaagccagactgtcaaaaaaagggcacatgtcactttgcaaaggaatgtattaactcctctcccagggtcaacttagtctacgtgtcttttgtataacattaatttccaccagatctactagatgttcagtcatgtcctttcaggtcctgaaggcaggctcactctctgatgcatctttttatatcatggtgggtgtgaagtgaaaagaggagacacagaaatatgcacaaacccacaattagtccatatttagaaaactttctgtgggttcaagcatttacacagagatgattttatctcatttctccattaatttcccatttgaaatgaaaaccagctaattctaaattctaaagccctgggggaaaccttccaggctttgtctatcagacagactttgtcataaaaaacacagaaaaacaaaaataaaacattacgctggaatcagcttttgagagtttgtgctttaaaaacacagtgcctaacagcaccaagcatatcatagatgctcaataaatatttgtagatttattaagagtaataacatggtgtttaaagaaccaaccaccattttgtaaaataggcaaaactacattaatttctttcacctgatttgataaagcagtgtggagcaatgaatgagagaatctgcaaattaaatatgaactctaatttgattgcagagagaaaattactgagaactttgcaaaaaacattgccacagtagccttgacactcaacagtgcaacgaagagttaatgtttccactgcaatatgaactggttcccacagctcttaggagatagagtgtaatcacttaaatgggaaatgaactctaattccacttgagaaaaggtatgttatgttcataattttatctgaaaattattaatatatttcagggagatggtcctctcattcagcatccctcaaagtaatgcaggcataagtatcaggggaccttgttatataacttcagtacagcattgtcttatacaagtgttctctcttccacatctgtagtagctgctttctaatattgtagatttttacagttgtgacacccctgggatgacagacatgagaatatggaggattaaaggttacaaaacttaaacaaaaaagggaagctcctctatgttatgtgaaaaccccttacaaaaggcagtttattgacaaataaatgctttatacattcaggtttttcccatctctcaatagtgatggtttccaaagaagaaactcagtagtgaagaatacatacttttttttttttgcattagtttgatcagttgaaaatcagaaccttcaaagcatcttgtgaatgagagaaatggaactggacctgggcaaggcatggggatggtagagatccatatgaataaatgatttagctgttgatgtggacagcaagagagttggtgggaaatgttacagcagacctgaccacgctacaaagggtctgtgaagaacacagtacaggtatcaaaacaccaaaacaaaactaaactaaaaacaagaacaaactgcaactttgccaaactgtaaacaaggtaaagcatttcacaggttcaaagttcaagggaagtaaacgtctttaaattatttttgtcagttcaaccctgatttaaaaatatggctagcaaaaacaaggaagccacagctgtcgacatcctgagcaagcatcggtctcctttgagaagctgcactcccaagcctcttctcaagctgctacacgaggaggagacacttctctcttgaattccatctcagttctctttatttccacactcttggaatacatcgattgctttccattttggtgtctacagttctggctgctatagatttagacgtggggatactggaggagggaaggcaaattctcggaggatgctccgggcaacttcgacattattctgggctatctctaaggctctcttcacctcttcaaaggcataaccctctcccatgagttttgcaatttttgcatcgacattttccaatgccgcctcaggcccatggggttttctgtggtgaatttctggtgcagtcctgcgcggtcgtggtttagggggtctggctggtgcctgtgaaccatctgaacatgaaggaagctgatcatagtcctgtgatgttctgttagttttgacattttcacctggtaaccttctagcaggaggcaaaggaacttggccacttgctagatcaacaaagggatctgaaggaagaagaaaaagatcctgtcctgaggatggccggctactggagccaggaggttttgaatgttcaatgagactatgccttgcaggaggtgggggaggtgggagagatggagggagggcatcaaaagcatcttcaccctttaaatatatgcttaagtcagggatgtttgatttcttctctgaagatggaccatgtgttccattcagcatacagtgaccattatcacaagactttatgctagggaggagggtggtaactggaggaggaggagaaagccggggaggaacatcatattcttcacttccaaggtgaccattggaaaagaccttagctccttctaaaggcaaatcatggcgtctgtgtttccgcataagcactgggtcagagcccactctactgtgccttccattgacatttgaactcgctgtgattccaggttttggagagccctcccctaggagtcgacatcccacaagctgattagtcccaaacacatcccgagggcaccatgcttcaagaggcattggcgggtctctggaaggcacgctttccacatgatggatgtgtctactcagtctattgtctggtgggattggtggaggtctttcaggtggcggtggaggaggatctcttaagggaggaggtggtgctgggagtggtttatcttgttttctcaccatgcaaggagaagactttggtgaacccgttgggctgccacagggagatctaactatgcctttctgaattagatccaggcgaggaggcacgggtggcaggcttagatgtgggatctggagtgggtcaggctgtggctttcttctctgggcaaggggagaggatcctggtgatgtgactggtgagttctgcctgtcagtgcactttcggacgtttgccaaccgattcatcatcaaggactcctcacgatcatcatcgtcgtccaagtctagcatcggcatgccaaaggggtcaatgatgctgcaacacctggagccttcatctcttggatcaaaggggtccacgattatgggctcagttccttttatttcacaacgacagaaagggcagccctgaccatccgactcctgccatgccgtaaggcaagaggtgcacatcaaatgcccacaaggctcaatcttgacatctttgtcattctctgcacaaatcttacagagctgaaaagtggagcccatttcacaatataattcatattgttcctgtgtaacttttatatggtcatgaggtgtaggttcacataatccagttaaatcaggattataactcctcccatcaggataaagataaaatccttccctgctgccatcaatcagggcttgaaataagggcttgttatgaggtatggtctgtaagatattcccatccccagtcacatagccaatggcccactgtcccaatcgagtgcaacttaaccggaaaatatagcttccgggtttggtgctatatttctgtagtcgtgctttaacttcatcatatgtgagaaatgccatgtaacctggatgtgtcacagctaagaaattccaattccgcaaaatagagccccaaggctgaaacagcctggtaaaaatatcaaattcaaaaactgaaatgtaatcattgcaagttaaatcaattgttgattttagagccattgcttccaggccagagctaatctggtggacctcatgaaggcactgtctgaatactttccatggtacgatagttttgtctccaaaaaactttctccagaattcagcagcatctgcttttgtgatacgaaagttatctccctggaattgaccattgggaaagattgctttgatttctgccagcatgtgactgaagataagggacagttttgtgagatttcgtctgtcctgtgactgttcttcatacattctctccttgccttctttaaagagtcttattgcccgttttgactttttcataaggctatcaatgtagattttaaagtactcattctcactgagttgggcaagtttctggttgtcatcatatttactcaatataagtcgtaaatgctgatatgtatcaggcaaaatatcaagtatatatggtgggctatttttcaactgaagtttgggattttggcacagtcttaccactttgtccatgagcttccaagtcttctccacggtcctgcgatctgcggcagcttgcttagggggtccaactgcatcctgaatagcatcaataatacccaaaattcgaccttttcggggatttcctcctcgaccaccagggtttctgccattcattgagtttgccatctggaattttagttcgtcaagacaaatccacacccgctctcccctcccgcccgactcggggaggccgcgggacgccgcagcagcactagcaggaggaggagaccgctcgctggac

SEQ ID NO: 9412 - RNA, 5633 nt, Homo sapiens
  source 1..5633: mol_type = other RNA
aggaggcatcttgagaaatggaaggaatgtctaactttttggatcacagtgaaacaaagtctggatcacttccagacatcaacgagcagtcgcttttacaataaaaaaaaatttttttaggtttaatttcataggtgatagatagcaatgggtctttcttgacagtgtttaatagaaagttttcctcttttcattccattacgtatgaatttttgattcattctttttaaatgacaatactaatggttgctattgagtacaagatgcagagattttgctggaggctggtaaattttctctgcaaaacagatatccccccaccccccacccccaaatttcaggtccaggtttgctatatcatcactagtccttttttaattctcactggaaattttcaaatattgtttataaactgaatgagaatgtgctatgttctctaacattcttattttacatcattctctaatatattaggaatgttgcaacaatgttatcacaatgaagtggcaacttttggcctttagactgtacctatcatcagcaatcataaaaaggccaaaataaacagtgctattccaaggtgacatctgaaactgttaaaacaagtgaaaaatcataatgacaaaacaggggttcataaagcaaaagaaaatttgccaatgcaattttaaaagtgtaagaaacttcactcatgtacctactcatgggaagaacatctaaggcaaatgaaaaattcccctccagggacataaccagctcagaaccatctgaaaaaattcatacaaaagcagaaattacccaaggcctgtgagtcctcatctcataccatgaaagccagactgtcaaaaaaagggcacatgtcactttgcaaaggaatgtattaactcctctcccagggtcaacttagtctacgtgtcttttgtataacattaatttccaccagatctactagatgttcagtcatgtcctttcaggtcctgaaggcaggctcactctctgatgcatctttttatatcatggtgggtgtgaagtgaaaagaggagacacagaaatatgcacaaacccacaattagtccatatttagaaaactttctgtgggttcaagcatttacacagagatgattttatctcatttctccattaatttcccatttgaaatgaaaaccagctaattctaaattctaaagccctgggggaaaccttccaggctttgtctatcagacagactttgtcataaaaaacacagaaaaacaaaaataaaacattacgctggaatcagcttttgagagtttgtgctttaaaaacacagtgcctaacagcaccaagcatatcatagatgctcaataaatatttgtagatttattaagagtaataacatggtgtttaaagaaccaaccaccattttgtaaaataggcaaaactacattaatttctttcacctgatttgataaagcagtgtggagcaatgaatgagagaatctgcaaattaaatatgaactctaatttgattgcagagagaaaattactgagaactttgcaaaaaacattgccacagtagccttgacactcaacagtgcaacgaagagttaatgtttccactgcaatatgaactggttcccacagctcttaggagatagagtgtaatcacttaaatgggaaatgaactctaattccacttgagaaaaggtatgttatgttcataattttatctgaaaattattaatatatttcagggagatggtcctctcattcagcatccctcaaagtaatgcaggcataagtatcaggggaccttgttatataacttcagtacagcattgtcttatacaagtgttctctcttccacatctgtagtagctgctttctaatattgtagatttttacagttgtgacacccctgggatgacagacatgagaatatggaggattaaaggttacaaaacttaaacaaaaaagggaagctcctctatgttatgtgaaaaccccttacaaaaggcagtttattgacaaataaatgctttatacattcaggtttttcccatctctcaatagtgatggtttccaaagaagaaactcagtagtgaagaatacatacttttttttttttgcattagtttgatcagttgaaaatcagaaccttcaaagcatcttgtgaatgagagaaatggaactggacctgggcaaggcatggggatggtagagatccatatgaataaatgatttagctgttgatgtggacagcaagagagttggtgggaaatgttacagcagacctgaccacgctacaaagggtctgtgaagaacacagtacaggtatcaaaacaccaaaacaaaactaaactaaaaacaagaacaaactgcaactttgccaaactgtaaacaaggtaaagcatttcacaggttcaaagttcaagggaagtaaacgtctttaaattatttttgtcagttcaaccctgatttaaaaatatggctagcaaaaacaaggaagccacagctgtcgacatcctgagcaagcatcggtctcctttgagaagctgcactcccaagcctcttctcaagctgctacacgaggaggagacacttctctcttgaattccatctcagttctctttatttccacactcttggaatacatcgattgctttccattttggtgtctacagttctggctgctatagatttagacgtggggatactggaggagggaaggcaaattctcggaggatgctccgggcaacttcgacattattctgggctatctctaaggctctcttcacctcttcaaaggcataaccctctcccatgagttttgcaatttttgcatcgacattttccaatgccgcctcaggcccatggggttttctgtggtgaatttctggtgcagtcctgcgcggtcgtggtttagggggtctggctggtgcctgtgaaccatctgaacatgaaggaagctgatcatagtcctgtgatgttctgttagttttgacattttcacctggtaaccttctagcaggaggcaaaggaacttggccacttgctagatcaacaaagggatctgaaggaagaagaaaaagatcctgtcctgaggatggccggctactggagccaggaggttttgaatgttcaatgagactatgccttgcaggaggtgggggaggtgggagagatggagggagggcatcaaaagcatcttcaccctttaaatatatgcttaagtcagggatgtttgatttcttctctgaagatggaccatgtgttccattcagcatacagtgaccattatcacaagactttatgctagggaggagggtggtaactggaggaggaggagaaagccggggaggaacatcatattcttcacttccaaggtgaccattggaaaagaccttagctccttctaaaggcaaatcatggcgtctgtgtttccgcataagcactgggtcagagcccactctactgtgccttccattgacatttgaactcgctgtgattccaggttttggagagccctcccctaggagtcgacatcccacaagctgattagtcccaaacacatcccgagggcaccatgcttcaagaggcattggcgggtctctggaaggcacgctttccacatgatggatgtgtctactcagtctattgtctggtgggattggtggaggtctttcaggtggcggtggaggaggatctcttaagggaggaggtggtgctgggagtggtttatcttgttttctcaccatgcaaggagaagactttggtgaacccgttgggctgccacagggagatctaactatgcctttctgaattagatccaggcgaggaggcacgggtggcaggcttagatgtgggatctggagtgggtcaggctgtggctttcttctctgggcaaggggagaggatcctggtgatgtgactggtgagttctgcctgtcagtgcactttcggacgtttgccaaccgattcatcatcaaggactcctcacgatcatcatcgtcgtccaagtctagcatcggcatgccaaaggggtcaatgatgctgcaacacctggagccttcatctcttggatcaaaggggtccacgattatgggctcagttccttttatttcacaacgacagaaagggcagccctgaccatccgactcctgccatgccgtaaggcaagaggtgcacatcaaatgcccacaaggctcaatcttgacatctttgtcattctctgcacaaatcttacagagctgaaaagtggagcccatttcacaatataattcatattgttcctgtgtaacttttatatggtcatgaggtgtaggttcacataatccagttaaatcaggattataactcctcccatcaggataaagataaaatccttccctgctgccatcaatcagggcttgaaataagggcttgttatgaggtatggtctgtaagatattcccatccccagtcacatagccaatggcccactgtcccaatcgagtgcaacttaaccggaaaatatagcttccgggtttggtgctatatttctgtagtcgtgctttaacttcatcatatgtgagaaatgccatgtaacctggatgtgtcacagctaagaaattccaattccgcaaaatagagccccaaggctgaaacagcctggtaaaaatatcaaattcaaaaactgaaatgtaatcattgcaagttaaatcaattgttgattttagagccattgcttccaggccagagctaatctggtggacctcatgaaggcactgtctgaatactttccatggtacgatagttttgtctccaaaaaactttctccagaattcagcagcatctgcttttgtgatacgaaagttatctccctggaattgaccattgggaaagattgctttgatttctgccagcatgtgactgaagataagggacagttttgtgagatttcgtctgtcctgtgactgttcttcatacattctctccttgccttctttaaagagtcttattgcccgttttgactttttcataaggctatcaatgtagattttaaagtactcattctcactgagttgggcaagtttctggttgtcatcatatttactcaatataagtcgtaaatgctgatatgtatcaggcaaaatatcaagtatatatggtgggctatttttcaactgaagtttgggattttggcacagtcttaccactttgtccatgagcttccaagtcttctccacggtcctgcgatctgcggcagcttgcttagggggtccaactgcatcctgaatagcatcaataatacccaaaattcgaccttttcggggatttcctcctcgaccaccagggtttctgccattcattgagtttgccatctggaattttagttctttcggcgccgtagctgtccagagacacgcgtgtgcgcgggtcccactccacacgcacgcagcccagtgtgtgtggggagccccggctgggagtgggatcgctgagaacagctcgctcccgaagaaggagcaacccagcgcgcaggcctccgagacgtggaaacgcaacaattaccgtcaagacaaatccacacccgctctcccctcccgcccgactcggggaggccgcgggacgccgcagcagcactagcaggaggaggagaccgctcgctggac

SEQ ID NO: 9413 - RNA, 5476 nt, Homo sapiens
  source 1..5476: mol_type = other RNA
aggaggcatcttgagaaatggaaggaatgtctaactttttggatcacagtgaaacaaagtctggatcacttccagacatcaacgagcagtcgcttttacaataaaaaaaaatttttttaggtttaatttcataggtgatagatagcaatgggtctttcttgacagtgtttaatagaaagttttcctcttttcattccattacgtatgaatttttgattcattctttttaaatgacaatactaatggttgctattgagtacaagatgcagagattttgctggaggctggtaaattttctctgcaaaacagatatccccccaccccccacccccaaatttcaggtccaggtttgctatatcatcactagtccttttttaattctcactggaaattttcaaatattgtttataaactgaatgagaatgtgctatgttctctaacattcttattttacatcattctctaatatattaggaatgttgcaacaatgttatcacaatgaagtggcaacttttggcctttagactgtacctatcatcagcaatcataaaaaggccaaaataaacagtgctattccaaggtgacatctgaaactgttaaaacaagtgaaaaatcataatgacaaaacaggggttcataaagcaaaagaaaatttgccaatgcaattttaaaagtgtaagaaacttcactcatgtacctactcatgggaagaacatctaaggcaaatgaaaaattcccctccagggacataaccagctcagaaccatctgaaaaaattcatacaaaagcagaaattacccaaggcctgtgagtcctcatctcataccatgaaagccagactgtcaaaaaaagggcacatgtcactttgcaaaggaatgtattaactcctctcccagggtcaacttagtctacgtgtcttttgtataacattaatttccaccagatctactagatgttcagtcatgtcctttcaggtcctgaaggcaggctcactctctgatgcatctttttatatcatggtgggtgtgaagtgaaaagaggagacacagaaatatgcacaaacccacaattagtccatatttagaaaactttctgtgggttcaagcatttacacagagatgattttatctcatttctccattaatttcccatttgaaatgaaaaccagctaattctaaattctaaagccctgggggaaaccttccaggctttgtctatcagacagactttgtcataaaaaacacagaaaaacaaaaataaaacattacgctggaatcagcttttgagagtttgtgctttaaaaacacagtgcctaacagcaccaagcatatcatagatgctcaataaatatttgtagatttattaagagtaataacatggtgtttaaagaaccaaccaccattttgtaaaataggcaaaactacattaatttctttcacctgatttgataaagcagtgtggagcaatgaatgagagaatctgcaaattaaatatgaactctaatttgattgcagagagaaaattactgagaactttgcaaaaaacattgccacagtagccttgacactcaacagtgcaacgaagagttaatgtttccactgcaatatgaactggttcccacagctcttaggagatagagtgtaatcacttaaatgggaaatgaactctaattccacttgagaaaaggtatgttatgttcataattttatctgaaaattattaatatatttcagggagatggtcctctcattcagcatccctcaaagtaatgcaggcataagtatcaggggaccttgttatataacttcagtacagcattgtcttatacaagtgttctctcttccacatctgtagtagctgctttctaatattgtagatttttacagttgtgacacccctgggatgacagacatgagaatatggaggattaaaggttacaaaacttaaacaaaaaagggaagctcctctatgttatgtgaaaaccccttacaaaaggcagtttattgacaaataaatgctttatacattcaggtttttcccatctctcaatagtgatggtttccaaagaagaaactcagtagtgaagaatacatacttttttttttttgcattagtttgatcagttgaaaatcagaaccttcaaagcatcttgtgaatgagagaaatggaactggacctgggcaaggcatggggatggtagagatccatatgaataaatgatttagctgttgatgtggacagcaagagagttggtgggaaatgttacagcagacctgaccacgctacaaagggtctgtgaagaacacagtacaggtatcaaaacaccaaaacaaaactaaactaaaaacaagaacaaactgcaactttgccaaactgtaaacaaggtaaagcatttcacaggttcaaagttcaagggaagtaaacgtctttaaattatttttgtcagttcaaccctgatttaaaaatatggctagcaaaaacaaggaagccacagctgtcgacatcctgagcaagcatcggtctcctttgagaagctgcactcccaagcctcttctcaagctgctacacgaggaggagacacttctctcttgaattccatctcagttctctttatttccacactcttggaatacatcgattgctttccattttggtgtctacagttctggctgctatagatttagacgtggggatactggaggagggaaggcaaattctcggaggatgctccgggcaacttcgacattattctgggctatctctaaggctctcttcacctcttcaaaggcataaccctctcccatgagttttgcaatttttgcatcgacattttccaatgccgcctcaggcccatggggttttctgtggtgaatttctggtgcagtcctgcgcggtcgtggtttagggggtctggctggtgcctgtgaaccatctgaacatgaaggaagctgatcatagtcctgtgatgttctgttagttttgacattttcacctggtaaccttctagcaggaggcaaaggaacttggccacttgctagatcaacaaagggatctgaaggaagaagaaaaagatcctgtcctgaggatggccggctactggagccaggaggttttgaatgttcaatgagactatgccttgcaggaggtgggggaggtgggagagatggagggagggcatcaaaagcatcttcaccctttaaatatatgcttaagtcagggatgtttgatttcttctctgaagatggaccatgtgttccattcagcatacagtgaccattatcacaagactttatgctagggaggagggtggtaactggaggaggaggagaaagccggggaggaacatcatattcttcacttccaaggtgaccattggaaaagaccttagctccttctaaaggcaaatcatggcgtctgtgtttccgcataagcactgggtcagagcccactctactgtgccttccattgacatttgaactcgctgtgattccaggttttggagagccctcccctaggagtcgacatcccacaagctgattagtcccaaacacatcccgagggcaccatgcttcaagaggcattggcgggtctctggaaggcacgctttccacatgatggatgtgtctactcagtctattgtctggtgggattggtggaggtctttcaggtggcggtggaggaggatctcttaagggaggaggtggtgctgggagtggtttatcttgttttctcaccatgcaaggagaagactttggtgaacccgttgggctgccacagggagatctaactatgcctttctgaattagatccaggcgaggaggcacgggtggcaggcttagatgtgggatctggagtgggtcaggctgtggctttcttctctgggcaaggggagaggatcctggtgatgtgactggtgagttctgcctgtcagtgcactttcggacgtttgccaaccgattcatcatcaaggactcctcacgatcatcatcgtcgtccaagtctagcatcggcatgccaaaggggtcaatgatgctgcaacacctggagccttcatctcttggatcaaaggggtccacgattatgggctcagttccttttatttcacaacgacagaaagggcagccctgaccatccgactcctgccatgccgtaaggcaagaggtgcacatcaaatgcccacaaggctcaatcttgacatctttgtcattctctgcacaaatcttacagagctgaaaagtggagcccatttcacaatataattcatattgttcctgtgtaacttttatatggtcatgaggtgtaggttcacataatccagttaaatcaggattataactcctcccatcaggataaagataaaatccttccctgctgccatcaatcagggcttgaaataagggcttgttatgaggtatggtctgtaagatattcccatccccagtcacatagccaatggcccactgtcccaatcgagtgcaacttaaccggaaaatatagcttccgggtttggtgctatatttctgtagtcgtgctttaacttcatcatatgtgagaaatgccatgtaacctggatgtgtcacagctaagaaattccaattccgcaaaatagagccccaaggttgtctccaaaaaactttctccagaattcagcagcatctgcttttgtgatacgaaagttatctccctggaattgaccattgggaaagattgctttgatttctgccagcatgtgactgaagataagggacagttttgtgagatttcgtctgtcctgtgactgttcttcatacattctctccttgccttctttaaagagtcttattgcccgttttgactttttcataaggctatcaatgtagattttaaagtactcattctcactgagttgggcaagtttctggttgtcatcatatttactcaatataagtcgtaaatgctgatatgtatcaggcaaaatatcaagtatatatggtgggctatttttcaactgaagtttgggattttggcacagtcttaccactttgtccatgagcttccaagtcttctccacggtcctgcgatctgcggcagcttgcttagggggtccaactgcatcctgaatagcatcaataatacccaaaattcgaccttttcggggatttcctcctcgaccaccagggtttctgccattcattgagtttgccatctggaattttagttctttcggcgccgtagctgtccagagacacgcgtgtgcgcgggtcccactccacacgcacgcagcccagtgtgtgtggggagccccggctgggagtgggatcgctgagaacagctcgctcccgaagaaggagcaacccagcgcgcaggcctccgagacgtggaaacgcaacaattaccgtcaagacaaatccacacccgctctcccctcccgcccgactcggggaggccgcgggacgccgcagcagcactagcaggaggaggagaccgctcgctggac

SEQ ID NO: 9414 - RNA, 5962 nt, Homo sapiens
  source 1..5962: mol_type = other RNA
aggaggcatcttgagaaatggaaggaatgtctaactttttggatcacagtgaaacaaagtctggatcacttccagacatcaacgagcagtcgcttttacaataaaaaaaaatttttttaggtttaatttcataggtgatagatagcaatgggtctttcttgacagtgtttaatagaaagttttcctcttttcattccattacgtatgaatttttgattcattctttttaaatgacaatactaatggttgctattgagtacaagatgcagagattttgctggaggctggtaaattttctctgcaaaacagatatccccccaccccccacccccaaatttcaggtccaggtttgctatatcatcactagtccttttttaattctcactggaaattttcaaatattgtttataaactgaatgagaatgtgctatgttctctaacattcttattttacatcattctctaatatattaggaatgttgcaacaatgttatcacaatgaagtggcaacttttggcctttagactgtacctatcatcagcaatcataaaaaggccaaaataaacagtgctattccaaggtgacatctgaaactgttaaaacaagtgaaaaatcataatgacaaaacaggggttcataaagcaaaagaaaatttgccaatgcaattttaaaagtgtaagaaacttcactcatgtacctactcatgggaagaacatctaaggcaaatgaaaaattcccctccagggacataaccagctcagaaccatctgaaaaaattcatacaaaagcagaaattacccaaggcctgtgagtcctcatctcataccatgaaagccagactgtcaaaaaaagggcacatgtcactttgcaaaggaatgtattaactcctctcccagggtcaacttagtctacgtgtcttttgtataacattaatttccaccagatctactagatgttcagtcatgtcctttcaggtcctgaaggcaggctcactctctgatgcatctttttatatcatggtgggtgtgaagtgaaaagaggagacacagaaatatgcacaaacccacaattagtccatatttagaaaactttctgtgggttcaagcatttacacagagatgattttatctcatttctccattaatttcccatttgaaatgaaaaccagctaattctaaattctaaagccctgggggaaaccttccaggctttgtctatcagacagactttgtcataaaaaacacagaaaaacaaaaataaaacattacgctggaatcagcttttgagagtttgtgctttaaaaacacagtgcctaacagcaccaagcatatcatagatgctcaataaatatttgtagatttattaagagtaataacatggtgtttaaagaaccaaccaccattttgtaaaataggcaaaactacattaatttctttcacctgatttgataaagcagtgtggagcaatgaatgagagaatctgcaaattaaatatgaactctaatttgattgcagagagaaaattactgagaactttgcaaaaaacattgccacagtagccttgacactcaacagtgcaacgaagagttaatgtttccactgcaatatgaactggttcccacagctcttaggagatagagtgtaatcacttaaatgggaaatgaactctaattccacttgagaaaaggtatgttatgttcataattttatctgaaaattattaatatatttcagggagatggtcctctcattcagcatccctcaaagtaatgcaggcataagtatcaggggaccttgttatataacttcagtacagcattgtcttatacaagtgttctctcttccacatctgtagtagctgctttctaatattgtagatttttacagttgtgacacccctgggatgacagacatgagaatatggaggattaaaggttacaaaacttaaacaaaaaagggaagctcctctatgttatgtgaaaaccccttacaaaaggcagtttattgacaaataaatgctttatacattcaggtttttcccatctctcaatagtgatggtttccaaagaagaaactcagtagtgaagaatacatacttttttttttttgcattagtttgatcagttgaaaatcagaaccttcaaagcatcttgtgaatgagagaaatggaactggacctgggcaaggcatggggatggtagagatccatatgaataaatgatttagctgttgatgtggacagcaagagagttggtgggaaatgttacagcagacctgaccacgctacaaagggtctgtgaagaacacagtacaggtatcaaaacaccaaaacaaaactaaactaaaaacaagaacaaactgcaactttgccaaactgtaaacaaggtaaagcatttcacaggttcaaagttcaagggaagtaaacgtctttaaattatttttgtcagttcaaccctgatttaaaaatatggctagcaaaaacaaggaagccacagctgtcgacatcctgagcaagcatcggtctcctttgagaagctgcactcccaagcctcttctcaagctgctacacgaggaggagacacttctctcttgaattccatctcagttctctttatttccacactcttggaatacatcgattgctttccattttggtgtctacagttctggctgctatagatttagacgtggggatactggaggagggaaggcaaattctcggaggatgctccgggcaacttcgacattattctgggctatctctaaggctctcttcacctcttcaaaggcataaccctctcccatgagttttgcaatttttgcatcgacattttccaatgccgcctcaggcccatggggttttctgtggtgaatttctggtgcagtcctgcgcggtcgtggtttagggggtctggctggtgcctgtgaaccatctgaacatgaaggaagctgatcatagtcctgtgatgttctgttagttttgacattttcacctggtaaccttctagcaggaggcaaaggaacttggccacttgctagatcaacaaagggatctgaaggaagaagaaaaagatcctgtcctgaggatggccggctactggagccaggaggttttgaatgttcaatgagactatgccttgcaggaggtgggggaggtgggagagatggagggagggcatcaaaagcatcttcacctaatggagggatgagaagatcataatcagagggcgtcctgttgagtgaagaaccatgctttggattgtcccgagttggaggcctggcaggtggtaatggcacgggatcagaggctgaatcaaaaacatctccctttaaatatatgcttaagtcagggatgtttgatttcttctctgaagatggaccatgtgttccattcagcatacagtgaccattatcacaagaccgaacaggaggttttacattatgacaatgagatggttgtgaattcagggaaacagggtgggatgaaggaatcttgtattcatcatcatcttcctctactgggtctcttgttttctctgaaagagaatttgctaacggaccagtacactttatgctagggaggagggtggtaactggaggaggaggagaaagccggggaggaacatcatattcttcacttccaaggtgaccattggaaaagaccttagctccttctaaaggcaaatcatggcgtctgtgtttccgcataagcactgggtcagagcccactctactgtgccttccattgacatttgaactcgctgtgattccaggttttggagagccctcccctaggagtcgacatcccacaagctgattagtcccaaacacatcccgagggcaccatgcttcaagaggcattggcgggtctctggaaggcacgctttccacatgatggatgtgtctactcagtctattgtctggtgggattggtggaggtctttcaggtggcggtggaggaggatctcttaagggaggaggtggtgctgggagtggtttatcttgttttctcaccatgcaaggagaagactttggtgaacccgttgggctgccacagggagatctaactatgcctttctgaattagatccaggcgaggaggcacgggtggcaggcttagatgtgggatctggagtgggtcaggctgtggctttcttctctgggcaaggggagaggatcctggtgatgtgactggtgagttctgcctgtcagtgcactttcggacgtttgccaaccgattcatcatcaaggactcctcacgatcatcatcgtcgtccaagtctagcatcggcatgccaaaggggtcaatgatgctgcaacacctggagccttcatctcttggatcaaaggggtccacgattatgggctcagttccttttatttcacaacgacagaaagggcagccctgaccatccgactccaagaattttcaaagcacagtatctcccacagaaactcaataacttctggctgccatgccgtaaggcaagaggtgcacatcaaatgcccacaaggctcaatcttgacatctttgtcattctctgcacaaatcttacagagctgaaaagtggagcccatttcacaatataattcatattgttcctgtgtaacttttatatggtcatgaggtgtaggttcacataatccagttaaatcaggattataactcctcccatcaggataaagataaaatccttccctgctgccatcaatcagggcttgaaataagggcttgttatgaggtatggtctgtaagatattcccatccccagtcacatagccaatggcccactgtcccaatcgagtgcaacttaaccggaaaatatagcttccgggtttggtgctatatttctgtagtcgtgctttaacttcatcatatgtgagaaatgccatgtaacctggatgtgtcacagctaagaaattccaattccgcaaaatagagccccaaggctgaaacagcctggtaaaaatatcaaattcaaaaactgaaatgtaatcattgcaagttaaatcaattgttgattttagagccattgcttccaggccagagctaatctggtggacctcatgaaggcactgtctgaatactttccatggtacgatagttttgtctccaaaaaactttctccagaattcagcagcatctgcttttgtgatacgaaagttatctccctggaattgaccattgggaaagattgctttgatttctgccagcatgtgactgaagataagggacagttttgtgagatttcgtctgtcctgtgactgttcttcatacattctctccttgccttctttaaagagtcttattgcccgttttgactttttcataaggctatcaatgtagattttaaagtactcattctcactgagttgggcaagtttctggttgtcatcatatttactcaatataagtcgtaaatgctgatatgtatcaggcaaaatatcaagtatatatggtgggctatttttcaactgaagtttgggattttggcacagtcttaccactttgtccatgagcttccaagtcttctccacggtcctgcgatctgcggcagcttgcttagggggtccaactgcatcctgaatagcatcaataatacccaaaattcgaccttttcggggatttcctcctcgaccaccagggtttctgccattcattgagtttgccatctggaattttagttctttcggcgccgtagctgtccagagacacgcgtgtgcgcgggtcccactccacacgcacgcagcccagtgtgtgtggggagccccggctgggagtgggatcgctgagaacagctcgctcccgaagaaggagcaacccagcgcgcaggcctccgagacgtggaaacgcaacaattaccgtcaagacaaatccacacccgctctcccctcccgcccgactcggggaggccgcgggacgccgcagcagcactagcaggaggaggagaccgctcgctggac

SEQ ID NO: 9415 - RNA, 5566 nt, Homo sapiens
  source 1..5566: mol_type = other RNA
aggaggcatcttgagaaatggaaggaatgtctaactttttggatcacagtgaaacaaagtctggatcacttccagacatcaacgagcagtcgcttttacaataaaaaaaaatttttttaggtttaatttcataggtgatagatagcaatgggtctttcttgacagtgtttaatagaaagttttcctcttttcattccattacgtatgaatttttgattcattctttttaaatgacaatactaatggttgctattgagtacaagatgcagagattttgctggaggctggtaaattttctctgcaaaacagatatccccccaccccccacccccaaatttcaggtccaggtttgctatatcatcactagtccttttttaattctcactggaaattttcaaatattgtttataaactgaatgagaatgtgctatgttctctaacattcttattttacatcattctctaatatattaggaatgttgcaacaatgttatcacaatgaagtggcaacttttggcctttagactgtacctatcatcagcaatcataaaaaggccaaaataaacagtgctattccaaggtgacatctgaaactgttaaaacaagtgaaaaatcataatgacaaaacaggggttcataaagcaaaagaaaatttgccaatgcaattttaaaagtgtaagaaacttcactcatgtacctactcatgggaagaacatctaaggcaaatgaaaaattcccctccagggacataaccagctcagaaccatctgaaaaaattcatacaaaagcagaaattacccaaggcctgtgagtcctcatctcataccatgaaagccagactgtcaaaaaaagggcacatgtcactttgcaaaggaatgtattaactcctctcccagggtcaacttagtctacgtgtcttttgtataacattaatttccaccagatctactagatgttcagtcatgtcctttcaggtcctgaaggcaggctcactctctgatgcatctttttatatcatggtgggtgtgaagtgaaaagaggagacacagaaatatgcacaaacccacaattagtccatatttagaaaactttctgtgggttcaagcatttacacagagatgattttatctcatttctccattaatttcccatttgaaatgaaaaccagctaattctaaattctaaagccctgggggaaaccttccaggctttgtctatcagacagactttgtcataaaaaacacagaaaaacaaaaataaaacattacgctggaatcagcttttgagagtttgtgctttaaaaacacagtgcctaacagcaccaagcatatcatagatgctcaataaatatttgtagatttattaagagtaataacatggtgtttaaagaaccaaccaccattttgtaaaataggcaaaactacattaatttctttcacctgatttgataaagcagtgtggagcaatgaatgagagaatctgcaaattaaatatgaactctaatttgattgcagagagaaaattactgagaactttgcaaaaaacattgccacagtagccttgacactcaacagtgcaacgaagagttaatgtttccactgcaatatgaactggttcccacagctcttaggagatagagtgtaatcacttaaatgggaaatgaactctaattccacttgagaaaaggtatgttatgttcataattttatctgaaaattattaatatatttcagggagatggtcctctcattcagcatccctcaaagtaatgcaggcataagtatcaggggaccttgttatataacttcagtacagcattgtcttatacaagtgttctctcttccacatctgtagtagctgctttctaatattgtagatttttacagttgtgacacccctgggatgacagacatgagaatatggaggattaaaggttacaaaacttaaacaaaaaagggaagctcctctatgttatgtgaaaaccccttacaaaaggcagtttattgacaaataaatgctttatacattcaggtttttcccatctctcaatagtgatggtttccaaagaagaaactcagtagtgaagaatacatacttttttttttttgcattagtttgatcagttgaaaatcagaaccttcaaagcatcttgtgaatgagagaaatggaactggacctgggcaaggcatggggatggtagagatccatatgaataaatgatttagctgttgatgtggacagcaagagagttggtgggaaatgttacagcagacctgaccacgctacaaagggtctgtgaagaacacagtacaggtatcaaaacaccaaaacaaaactaaactaaaaacaagaacaaactgcaactttgccaaactgtaaacaaggtaaagcatttcacaggttcaaagttcaagggaagtaaacgtctttaaattatttttgtcagttcaaccctgatttaaaaatatggctagcaaaaacaaggaagccacagctgtcgacatcctgagcaagcatcggtctcctttgagaagctgcactcccaagcctcttctcaagctgctacacgaggaggagacacttctctcttgaattccatctcagttctctttatttccacactcttggaatacatcgattgctttccattttggtgtctacagttctggctgctatagatttagacgtggggatactggaggagggaaggcaaattctcggaggatgctccgggcaacttcgacattattctgggctatctctaaggctctcttcacctcttcaaaggcataaccctctcccatgagttttgcaatttttgcatcgacattttccaatgccgcctcaggcccatggggttttctgtggtgaatttctggtgcagtcctgcgcggtcgtggtttagggggtctggctggtgcctgtgaaccatctgaacatgaaggaagctgatcatagtcctgtgatgttctgttagttttgacattttcacctggtaaccttctagcaggaggcaaaggaacttggccacttgctagatcaacaaagggatctgaaggaagaagaaaaagatcctgtcctgaggatggccggctactggagccaggaggttttgaatgttcaatgagactatgccttgcaggaggtgggggaggtgggagagatggagggagggcatcaaaagcatcttcacctaatggagggatgagaagatcataatcagagggcgtcctgttgagtgaagaaccatgctttggattgtcccgagttggaggcctggcaggtggtaatggcacgggatcagaggctgaatcaaaaacatctccctttaaatatatgcttaagtcagggatgtttgatttcttctctgaagatggaccatgtgttccattcagcatacagtgaccattatcacaagaccgaacaggaggttttacattatgacaatgagatggttgtgaattcagggaaacagggtgggatgaaggaatcttgtattcatcatcatcttcctctactgggtctcttgttttctctgaaagagaatttgctaacggaccagtacactttatgctagggaggagggtggtaactggaggaggaggagaaagccggggaggaacatcatattcttcacttccaaggtgaccattggaaaagaccttagctccttctaaaggcaaatcatggcgtctgtgtttccgcataagcactgggtcagagcccactctactgtgccttccattgacatttgaactcgctgtgattccaggttttggagagccctcccctaggagtcgacatcccacaagctgattagtcccaaacacatcccgagggcaccatgcttcaagaggcattggcgggtctctggaaggcacgctttccacatgatggatgtgtctactcagtctattgtctggtgggattggtggaggtctttcaggtggcggtggaggaggatctcttaagggaggaggtggtgctgggagtggtttatcttgttttctcaccatgcaaggagaagactttggtgaacccgttgggctgccacagggagatctaactatgcctttctgaattagatccaggcgaggaggcacgggtggcaggcttagatgtgggatctggagtgggtcaggctgtggctttcttctctgggcaaggggagaggatcctggtgatgtgactggtgagttctgcctgtcagtgcactttcggacgtttgccaaccgattcatcatcaaggactcctcacgatcatcatcgtcgtccaagtctagcatcggcatgccaaaggggtcaatgatgctgcaacacctggagccttcatctcttggatcaaaggggtccacgattatgggctcagttccttttatttcacaacgacagaaagggcagccctgaccatccgactcctgccatgccgtaaggcaagaggtgcacatcaaatgcccacaaggctcaatcttgacatctttgtcattctctgcacaaatcttacagagctgaaaagtggagcccatttcacaatataattcatattgttcctgtgtaacttttatatggtcatgaggtgtaggttcacataatccagttaaatcaggattataactcctcccatcaggataaagataaaatccttccctgctgccatcaatcagggcttgaaataagggcttgttatgaggtatggtctgtaagatattcccatccccagtcacatagccaatggcccactgtcccaatcgagtgcaacttaaccggaaaatatagcttccgggtttggtgctatatttctgtagtcgtgctttaacttcatcatatgtgagaaatgccatgtaacctggatgtgtcacagctaagaaattccaattccgcaaaatagagccccaaggctgaaacagcctggtaaaaatatcaaattcaaaaactgaaatgtaatcattgcaagttaaatcaattgttgattttagagccattgcttccaggccagagctaatctggtggacctcatgaaggcactgtctgaatactttccatggtacgatagttctgtcctgtgactgttcttcatacattctctccttgccttctttaaagagtcttattgcccgttttgactttttcataaggctatcaatgtagattttaaagtactcattctcactgagttgggcaagtttctggttgtcatcatatttactcaatataagtcgtaaatgctgatatgtatcaggcaaaatatcaagtatatatggtgggctatttttcaactgaagtttgggattttggcacagtcttaccactttgtccatgagcttccaagtcttctccacggtcctgcgatctgcggcagcttgcttagggggtccaactgcatcctgaatagcatcaataatacccaaaattcgaccttttcggggatttcctcctcgaccaccagggtttctgccattcattgagtttgccatctggaattttagttcaataaggggtggcaggtgggcgtgagcgtcgggaccgggagccaaagccatctggggctgaaaggcgggacttcctg

SEQ ID NO: 9416 - RNA, 5589 nt, Homo sapiens
  source 1..5589: mol_type = other RNA
aggaggcatcttgagaaatggaaggaatgtctaactttttggatcacagtgaaacaaagtctggatcacttccagacatcaacgagcagtcgcttttacaataaaaaaaaatttttttaggtttaatttcataggtgatagatagcaatgggtctttcttgacagtgtttaatagaaagttttcctcttttcattccattacgtatgaatttttgattcattctttttaaatgacaatactaatggttgctattgagtacaagatgcagagattttgctggaggctggtaaattttctctgcaaaacagatatccccccaccccccacccccaaatttcaggtccaggtttgctatatcatcactagtccttttttaattctcactggaaattttcaaatattgtttataaactgaatgagaatgtgctatgttctctaacattcttattttacatcattctctaatatattaggaatgttgcaacaatgttatcacaatgaagtggcaacttttggcctttagactgtacctatcatcagcaatcataaaaaggccaaaataaacagtgctattccaaggtgacatctgaaactgttaaaacaagtgaaaaatcataatgacaaaacaggggttcataaagcaaaagaaaatttgccaatgcaattttaaaagtgtaagaaacttcactcatgtacctactcatgggaagaacatctaaggcaaatgaaaaattcccctccagggacataaccagctcagaaccatctgaaaaaattcatacaaaagcagaaattacccaaggcctgtgagtcctcatctcataccatgaaagccagactgtcaaaaaaagggcacatgtcactttgcaaaggaatgtattaactcctctcccagggtcaacttagtctacgtgtcttttgtataacattaatttccaccagatctactagatgttcagtcatgtcctttcaggtcctgaaggcaggctcactctctgatgcatctttttatatcatggtgggtgtgaagtgaaaagaggagacacagaaatatgcacaaacccacaattagtccatatttagaaaactttctgtgggttcaagcatttacacagagatgattttatctcatttctccattaatttcccatttgaaatgaaaaccagctaattctaaattctaaagccctgggggaaaccttccaggctttgtctatcagacagactttgtcataaaaaacacagaaaaacaaaaataaaacattacgctggaatcagcttttgagagtttgtgctttaaaaacacagtgcctaacagcaccaagcatatcatagatgctcaataaatatttgtagatttattaagagtaataacatggtgtttaaagaaccaaccaccattttgtaaaataggcaaaactacattaatttctttcacctgatttgataaagcagtgtggagcaatgaatgagagaatctgcaaattaaatatgaactctaatttgattgcagagagaaaattactgagaactttgcaaaaaacattgccacagtagccttgacactcaacagtgcaacgaagagttaatgtttccactgcaatatgaactggttcccacagctcttaggagatagagtgtaatcacttaaatgggaaatgaactctaattccacttgagaaaaggtatgttatgttcataattttatctgaaaattattaatatatttcagggagatggtcctctcattcagcatccctcaaagtaatgcaggcataagtatcaggggaccttgttatataacttcagtacagcattgtcttatacaagtgttctctcttccacatctgtagtagctgctttctaatattgtagatttttacagttgtgacacccctgggatgacagacatgagaatatggaggattaaaggttacaaaacttaaacaaaaaagggaagctcctctatgttatgtgaaaaccccttacaaaaggcagtttattgacaaataaatgctttatacattcaggtttttcccatctctcaatagtgatggtttccaaagaagaaactcagtagtgaagaatacatacttttttttttttgcattagtttgatcagttgaaaatcagaaccttcaaagcatcttgtgaatgagagaaatggaactggacctgggcaaggcatggggatggtagagatccatatgaataaatgatttagctgttgatgtggacagcaagagagttggtgggaaatgttacagcagacctgaccacgctacaaagggtctgtgaagaacacagtacaggtatcaaaacaccaaaacaaaactaaactaaaaacaagaacaaactgcaactttgccaaactgtaaacaaggtaaagcatttcacaggttcaaagttcaagggaagtaaacgtctttaaattatttttgtcagttcaaccctgatttaaaaatatggctagcaaaaacaaggaagccacagctgtcgacatcctgagcaagcatcggtctcctttgagaagctgcactcccaagcctcttctcaagctgctacacgaggaggagacacttctctcttgaattccatctcagttctctttatttccacactcttggaatacatcgattgctttccattttggtgtctacagttctggctgctatagatttagacgtggggatactggaggagggaaggcaaattctcggaggatgctccgggcaacttcgacattattctgggctatctctaaggctctcttcacctcttcaaaggcataaccctctcccatgagttttgcaatttttgcatcgacattttccaatgccgcctcaggcccatggggttttctgtggtgaatttctggtgcagtcctgcgcggtcgtggtttagggggtctggctggtgcctgtgaaccatctgaacatgaaggaagctgatcatagtcctgtgatgttctgttagttttgacattttcacctggtaaccttctagcaggaggcaaaggaacttggccacttgctagatcaacaaagggatctgaaggaagaagaaaaagatcctgtcctgaggatggccggctactggagccaggaggttttgaatgttcaatgagactatgccttgcaggaggtgggggaggtgggagagatggagggagggcatcaaaagcatcttcacctaatggagggatgagaagatcataatcagagggcgtcctgttgagtgaagaaccatgctttggattgtcccgagttggaggcctggcaggtggtaatggcacgggatcagaggctgaatcaaaaacatctccctttaaatatatgcttaagtcagggatgtttgatttcttctctgaagatggaccatgtgttccattcagcatacagtgaccattatcacaagaccgaacaggaggttttacattatgacaatgagatggttgtgaattcagggaaacagggtgggatgaaggaatcttgtattcatcatcatcttcctctactgggtctcttgttttctctgaaagagaatttgctaacggaccagtacactttatgctagggaggagggtggtaactggaggaggaggagaaagccggggaggaacatcatattcttcacttccaaggtgaccattggaaaagaccttagctccttctaaaggcaaatcatggcgtctgtgtttccgcataagcactgggtcagagcccactctactgtgccttccattgacatttgaactcgctgtgattccaggttttggagagccctcccctaggagtcgacatcccacaagctgattagtcccaaacacatcccgagggcaccatgcttcaagaggcattggcgggtctctggaaggcacgctttccacatgatggatgtgtctactcagtctattgtctggtgggattggtggaggtctttcaggtggcggtggaggaggatctcttaagggaggaggtggtgctgggagtggtttatcttgttttctcaccatgcaaggagaagactttggtgaacccgttgggctgccacagggagatctaactatgcctttctgaattagatccaggcgaggaggcacgggtggcaggcttagatgtgggatctggagtgggtcaggctgtggctttcttctctgggcaaggggagaggatcctggtgatgtgactggtgagttctgcctgtcagtgcactttcggacgtttgccaaccgattcatcatcaaggactcctcacgatcatcatcgtcgtccaagtctagcatcggcatgccaaaggggtcaatgatgctgcaacacctggagccttcatctcttggatcaaaggggtccacgattatgggctcagttccttttatttcacaacgacagaaagggcagccctgaccatccgactcctgccatgccgtaaggcaagaggtgcacatcaaatgcccacaaggctcaatcttgacatctttgtcattctctgcacaaatcttacagagctgaaaagtggagcccatttcacaatataattcatattgttcctgtgtaacttttatatggtcatgaggtgtaggttcacataatccagttaaatcaggattataactcctcccatcaggataaagataaaatccttccctgctgccatcaatcagggcttgaaataagggcttgttatgaggtatggtctgtaagatattcccatccccagtcacatagccaatggcccactgtcccaatcgagtgcaacttaaccggaaaatatagcttccgggtttggtgctatatttctgtagtcgtgctttaacttcatcatatgtgagaaatgccatgtaacctggatgtgtcacagctaagaaattccaattccgcaaaatagagccccaaggctgaaacagcctggtaaaaatatcaaattcaaaaactgaaatgtaatcattgcaagttaaatcaattgttgattttagagccattgcttccaggccagagctaatctggtggacctcatgaaggcactgtctgaatactttccatggtacgatagttctgtcctgtgactgttcttcatacattctctccttgccttctttaaagagtcttattgcccgttttgactttttcataaggctatcaatgtagattttaaagtactcattctcactgagttgggcaagtttctggttgtcatcatatttactcaatataagtcgtaaatgctgatatgtatcaggcaaaatatcaagtatatatggtgggctatttttcaactgaagtttgggattttggcacagtcttaccactttgtccatgagcttccaagtcttctccacggtcctgcgatctgcggcagcttgcttagggggtccaactgcatcctgaatagcatcaataatacccaaaattcgaccttttcggggatttcctcctcgaccaccagggtttctgccattcattgagtttgccatctggaattttagttcgtcaagacaaatccacacccgctctcccctcccgcccgactcggggaggccgcgggacgccgcagcagcactagcaggaggaggagaccgctcgctggac

SEQ ID NO: 9417 - RNA, 5791 nt, Homo sapiens
  source 1..5791: mol_type = other RNA
aggaggcatcttgagaaatggaaggaatgtctaactttttggatcacagtgaaacaaagtctggatcacttccagacatcaacgagcagtcgcttttacaataaaaaaaaatttttttaggtttaatttcataggtgatagatagcaatgggtctttcttgacagtgtttaatagaaagttttcctcttttcattccattacgtatgaatttttgattcattctttttaaatgacaatactaatggttgctattgagtacaagatgcagagattttgctggaggctggtaaattttctctgcaaaacagatatccccccaccccccacccccaaatttcaggtccaggtttgctatatcatcactagtccttttttaattctcactggaaattttcaaatattgtttataaactgaatgagaatgtgctatgttctctaacattcttattttacatcattctctaatatattaggaatgttgcaacaatgttatcacaatgaagtggcaacttttggcctttagactgtacctatcatcagcaatcataaaaaggccaaaataaacagtgctattccaaggtgacatctgaaactgttaaaacaagtgaaaaatcataatgacaaaacaggggttcataaagcaaaagaaaatttgccaatgcaattttaaaagtgtaagaaacttcactcatgtacctactcatgggaagaacatctaaggcaaatgaaaaattcccctccagggacataaccagctcagaaccatctgaaaaaattcatacaaaagcagaaattacccaaggcctgtgagtcctcatctcataccatgaaagccagactgtcaaaaaaagggcacatgtcactttgcaaaggaatgtattaactcctctcccagggtcaacttagtctacgtgtcttttgtataacattaatttccaccagatctactagatgttcagtcatgtcctttcaggtcctgaaggcaggctcactctctgatgcatctttttatatcatggtgggtgtgaagtgaaaagaggagacacagaaatatgcacaaacccacaattagtccatatttagaaaactttctgtgggttcaagcatttacacagagatgattttatctcatttctccattaatttcccatttgaaatgaaaaccagctaattctaaattctaaagccctgggggaaaccttccaggctttgtctatcagacagactttgtcataaaaaacacagaaaaacaaaaataaaacattacgctggaatcagcttttgagagtttgtgctttaaaaacacagtgcctaacagcaccaagcatatcatagatgctcaataaatatttgtagatttattaagagtaataacatggtgtttaaagaaccaaccaccattttgtaaaataggcaaaactacattaatttctttcacctgatttgataaagcagtgtggagcaatgaatgagagaatctgcaaattaaatatgaactctaatttgattgcagagagaaaattactgagaactttgcaaaaaacattgccacagtagccttgacactcaacagtgcaacgaagagttaatgtttccactgcaatatgaactggttcccacagctcttaggagatagagtgtaatcacttaaatgggaaatgaactctaattccacttgagaaaaggtatgttatgttcataattttatctgaaaattattaatatatttcagggagatggtcctctcattcagcatccctcaaagtaatgcaggcataagtatcaggggaccttgttatataacttcagtacagcattgtcttatacaagtgttctctcttccacatctgtagtagctgctttctaatattgtagatttttacagttgtgacacccctgggatgacagacatgagaatatggaggattaaaggttacaaaacttaaacaaaaaagggaagctcctctatgttatgtgaaaaccccttacaaaaggcagtttattgacaaataaatgctttatacattcaggtttttcccatctctcaatagtgatggtttccaaagaagaaactcagtagtgaagaatacatacttttttttttttgcattagtttgatcagttgaaaatcagaaccttcaaagcatcttgtgaatgagagaaatggaactggacctgggcaaggcatggggatggtagagatccatatgaataaatgatttagctgttgatgtggacagcaagagagttggtgggaaatgttacagcagacctgaccacgctacaaagggtctgtgaagaacacagtacaggtatcaaaacaccaaaacaaaactaaactaaaaacaagaacaaactgcaactttgccaaactgtaaacaaggtaaagcatttcacaggttcaaagttcaagggaagtaaacgtctttaaattatttttgtcagttcaaccctgatttaaaaatatggctagcaaaaacaaggaagccacagctgtcgacatcctgagcaagcatcggtctcctttgagaagctgcactcccaagcctcttctcaagctgctacacgaggaggagacacttctctcttgaattccatctcagttctctttatttccacactcttggaatacatcgattgctttccattttggtgtctacagttctggctgctatagatttagacgtggggatactggaggagggaaggcaaattctcggaggatgctccgggcaacttcgacattattctgggctatctctaaggctctcttcacctcttcaaaggcataaccctctcccatgagttttgcaatttttgcatcgacattttccaatgccgcctcaggcccatggggttttctgtggtgaatttctggtgcagtcctgcgcggtcgtggtttagggggtctggctggtgcctgtgaaccatctgaacatgaaggaagctgatcatagtcctgtgatgttctgttagttttgacattttcacctggtaaccttctagcaggaggcaaaggaacttggccacttgctagatcaacaaagggatctgaaggaagaagaaaaagatcctgtcctgaggatggccggctactggagccaggaggttttgaatgttcaatgagactatgccttgcaggaggtgggggaggtgggagagatggagggagggcatcaaaagcatcttcacctaatggagggatgagaagatcataatcagagggcgtcctgttgagtgaagaaccatgctttggattgtcccgagttggaggcctggcaggtggtaatggcacgggatcagaggctgaatcaaaaacatctccctttaaatatatgcttaagtcagggatgtttgatttcttctctgaagatggaccatgtgttccattcagcatacagtgaccattatcacaagaccgaacaggaggttttacattatgacaatgagatggttgtgaattcagggaaacagggtgggatgaaggaatcttgtattcatcatcatcttcctctactgggtctcttgttttctctgaaagagaatttgctaacggaccagtacactttatgctagggaggagggtggtaactggaggaggaggagaaagccggggaggaacatcatattcttcacttccaaggtgaccattggaaaagaccttagctccttctaaaggcaaatcatggcgtctgtgtttccgcataagcactgggtcagagcccactctactgtgccttccattgacatttgaactcgctgtgattccaggttttggagagccctcccctaggagtcgacatcccacaagctgattagtcccaaacacatcccgagggcaccatgcttcaagaggcattggcgggtctctggaaggcacgctttccacatgatggatgtgtctactcagtctattgtctggtgggattggtggaggtctttcaggtggcggtggaggaggatctcttaagggaggaggtggtgctgggagtggtttatcttgttttctcaccatgcaaggagaagactttggtgaacccgttgggctgccacagggagatctaactatgcctttctgaattagatccaggcgaggaggcacgggtggcaggcttagatgtgggatctggagtgggtcaggctgtggctttcttctctgggcaaggggagaggatcctggtgatgtgactggtgagttctgcctgtcagtgcactttcggacgtttgccaaccgattcatcatcaaggactcctcacgatcatcatcgtcgtccaagtctagcatcggcatgccaaaggggtcaatgatgctgcaacacctggagccttcatctcttggatcaaaggggtccacgattatgggctcagttccttttatttcacaacgacagaaagggcagccctgaccatccgactcctgccatgccgtaaggcaagaggtgcacatcaaatgcccacaaggctcaatcttgacatctttgtcattctctgcacaaatcttacagagctgaaaagtggagcccatttcacaatataattcatattgttcctgtgtaacttttatatggtcatgaggtgtaggttcacataatccagttaaatcaggattataactcctcccatcaggataaagataaaatccttccctgctgccatcaatcagggcttgaaataagggcttgttatgaggtatggtctgtaagatattcccatccccagtcacatagccaatggcccactgtcccaatcgagtgcaacttaaccggaaaatatagcttccgggtttggtgctatatttctgtagtcgtgctttaacttcatcatatgtgagaaatgccatgtaacctggatgtgtcacagctaagaaattccaattccgcaaaatagagccccaaggctgaaacagcctggtaaaaatatcaaattcaaaaactgaaatgtaatcattgcaagttaaatcaattgttgattttagagccattgcttccaggccagagctaatctggtggacctcatgaaggcactgtctgaatactttccatggtacgatagttctgtcctgtgactgttcttcatacattctctccttgccttctttaaagagtcttattgcccgttttgactttttcataaggctatcaatgtagattttaaagtactcattctcactgagttgggcaagtttctggttgtcatcatatttactcaatataagtcgtaaatgctgatatgtatcaggcaaaatatcaagtatatatggtgggctatttttcaactgaagtttgggattttggcacagtcttaccactttgtccatgagcttccaagtcttctccacggtcctgcgatctgcggcagcttgcttagggggtccaactgcatcctgaatagcatcaataatacccaaaattcgaccttttcggggatttcctcctcgaccaccagggtttctgccattcattgagtttgccatctggaattttagttctttcggcgccgtagctgtccagagacacgcgtgtgcgcgggtcccactccacacgcacgcagcccagtgtgtgtggggagccccggctgggagtgggatcgctgagaacagctcgctcccgaagaaggagcaacccagcgcgcaggcctccgagacgtggaaacgcaacaattaccgtcaagacaaatccacacccgctctcccctcccgcccgactcggggaggccgcgggacgccgcagcagcactagcaggaggaggagaccgctcgctggacaccccacccctgtggcacacacagga

SEQ ID NO: 9418 - RNA, 5740 nt, Homo sapiens
  source 1..5740: mol_type = other RNA
aggaggcatcttgagaaatggaaggaatgtctaactttttggatcacagtgaaacaaagtctggatcacttccagacatcaacgagcagtcgcttttacaataaaaaaaaatttttttaggtttaatttcataggtgatagatagcaatgggtctttcttgacagtgtttaatagaaagttttcctcttttcattccattacgtatgaatttttgattcattctttttaaatgacaatactaatggttgctattgagtacaagatgcagagattttgctggaggctggtaaattttctctgcaaaacagatatccccccaccccccacccccaaatttcaggtccaggtttgctatatcatcactagtccttttttaattctcactggaaattttcaaatattgtttataaactgaatgagaatgtgctatgttctctaacattcttattttacatcattctctaatatattaggaatgttgcaacaatgttatcacaatgaagtggcaacttttggcctttagactgtacctatcatcagcaatcataaaaaggccaaaataaacagtgctattccaaggtgacatctgaaactgttaaaacaagtgaaaaatcataatgacaaaacaggggttcataaagcaaaagaaaatttgccaatgcaattttaaaagtgtaagaaacttcactcatgtacctactcatgggaagaacatctaaggcaaatgaaaaattcccctccagggacataaccagctcagaaccatctgaaaaaattcatacaaaagcagaaattacccaaggcctgtgagtcctcatctcataccatgaaagccagactgtcaaaaaaagggcacatgtcactttgcaaaggaatgtattaactcctctcccagggtcaacttagtctacgtgtcttttgtataacattaatttccaccagatctactagatgttcagtcatgtcctttcaggtcctgaaggcaggctcactctctgatgcatctttttatatcatggtgggtgtgaagtgaaaagaggagacacagaaatatgcacaaacccacaattagtccatatttagaaaactttctgtgggttcaagcatttacacagagatgattttatctcatttctccattaatttcccatttgaaatgaaaaccagctaattctaaattctaaagccctgggggaaaccttccaggctttgtctatcagacagactttgtcataaaaaacacagaaaaacaaaaataaaacattacgctggaatcagcttttgagagtttgtgctttaaaaacacagtgcctaacagcaccaagcatatcatagatgctcaataaatatttgtagatttattaagagtaataacatggtgtttaaagaaccaaccaccattttgtaaaataggcaaaactacattaatttctttcacctgatttgataaagcagtgtggagcaatgaatgagagaatctgcaaattaaatatgaactctaatttgattgcagagagaaaattactgagaactttgcaaaaaacattgccacagtagccttgacactcaacagtgcaacgaagagttaatgtttccactgcaatatgaactggttcccacagctcttaggagatagagtgtaatcacttaaatgggaaatgaactctaattccacttgagaaaaggtatgttatgttcataattttatctgaaaattattaatatatttcagggagatggtcctctcattcagcatccctcaaagtaatgcaggcataagtatcaggggaccttgttatataacttcagtacagcattgtcttatacaagtgttctctcttccacatctgtagtagctgctttctaatattgtagatttttacagttgtgacacccctgggatgacagacatgagaatatggaggattaaaggttacaaaacttaaacaaaaaagggaagctcctctatgttatgtgaaaaccccttacaaaaggcagtttattgacaaataaatgctttatacattcaggtttttcccatctctcaatagtgatggtttccaaagaagaaactcagtagtgaagaatacatacttttttttttttgcattagtttgatcagttgaaaatcagaaccttcaaagcatcttgtgaatgagagaaatggaactggacctgggcaaggcatggggatggtagagatccatatgaataaatgatttagctgttgatgtggacagcaagagagttggtgggaaatgttacagcagacctgaccacgctacaaagggtctgtgaagaacacagtacaggtatcaaaacaccaaaacaaaactaaactaaaaacaagaacaaactgcaactttgccaaactgtaaacaaggtaaagcatttcacaggttcaaagttcaagggaagtaaacgtctttaaattatttttgtcagttcaaccctgatttaaaaatatggctagcaaaaacaaggaagccacagctgtcgacatcctgagcaagcatcggtctcctttgagaagctgcactcccaagcctcttctcaagctgctacacgaggaggagacacttctctcttgaattccatctcagttctctttatttccacactcttggaatacatcgattgctttccattttggtgtctacagttctggctgctatagatttagacgtggggatactggaggagggaaggcaaattctcggaggatgctccgggcaacttcgacattattctgggctatctctaaggctctcttcacctcttcaaaggcataaccctctcccatgagttttgcaatttttgcatcgacattttccaatgccgcctcaggcccatggggttttctgtggtgaatttctggtgcagtcctgcgcggtcgtggtttagggggtctggctggtgcctgtgaaccatctgaacatgaaggaagctgatcatagtcctgtgatgttctgttagttttgacattttcacctggtaaccttctagcaggaggcaaaggaacttggccacttgctagatcaacaaagggatctgaaggaagaagaaaaagatcctgtcctgaggatggccggctactggagccaggaggttttgaatgttcaatgagactatgccttgcaggaggtgggggaggtgggagagatggagggagggcatcaaaagcatcttcacctaatggagggatgagaagatcataatcagagggcgtcctgttgagtgaagaaccatgctttggattgtcccgagttggaggcctggcaggtggtaatggcacgggatcagaggctgaatcaaaaacatctccctttaaatatatgcttaagtcagggatgtttgatttcttctctgaagatggaccatgtgttccattcagcatacagtgaccattatcacaagaccgaacaggaggttttacattatgacaatgagatggttgtgaattcagggaaacagggtgggatgaaggaatcttgtattcatcatcatcttcctctactgggtctcttgttttctctgaaagagaatttgctaacggaccagtacactttatgctagggaggagggtggtaactggaggaggaggagaaagccggggaggaacatcatattcttcacttccaaggtgaccattggaaaagaccttagctccttctaaaggcaaatcatggcgtctgtgtttccgcataagcactgggtcagagcccactctactgtgccttccattgacatttgaactcgctgtgattccaggttttggagagccctcccctaggagtcgacatcccacaagctgattagtcccaaacacatcccgagggcaccatgcttcaagaggcattggcgggtctctggaaggcacgctttccacatgatggatgtgtctactcagtctattgtctggtgggattggtggaggtctttcaggtggcggtggaggaggatctcttaagggaggaggtggtgctgggagtggtttatcttgttttctcaccatgcaaggagaagactttggtgaacccgttgggctgccacagggagatctaactatgcctttctgaattagatccaggcgaggaggcacgggtggcaggcttagatgtgggatctggagtgggtcaggctgtggctttcttctctgggcaaggggagaggatcctggtgatgtgactggtgagttctgcctgtcagtgcactttcggacgtttgccaaccgattcatcatcaaggactcctcacgatcatcatcgtcgtccaagtctagcatcggcatgccaaaggggtcaatgatgctgcaacacctggagccttcatctcttggatcaaaggggtccacgattatgggctcagttccttttatttcacaacgacagaaagggcagccctgaccatccgactcctgccatgccgtaaggcaagaggtgcacatcaaatgcccacaaggctcaatcttgacatctttgtcattctctgcacaaatcttacagagctgaaaagtggagcccatttcacaatataattcatattgttcctgtgtaacttttatatggtcatgaggtgtaggttcacataatccagttaaatcaggattataactcctcccatcaggataaagataaaatccttccctgctgccatcaatcagggcttgaaataagggcttgttatgaggtatggtctgtaagatattcccatccccagtcacatagccaatggcccactgtcccaatcgagtgcaacttaaccggaaaatatagcttccgggtttggtgctatatttctgtagtcgtgctttaacttcatcatatgtgagaaatgccatgtaacctggatgtgtcacagctaagaaattccaattccgcaaaatagagccccaaggctgaaacagcctggtaaaaatatcaaattcaaaaactgaaatgtaatcattgcaagttaaatcaattgttgattttagagccattgcttccaggccagagctaatctggtggacctcatgaaggcactgtctgaatactttccatggtacgatagttctgtcctgtgactgttcttcatacattctctccttgccttctttaaagagtcttattgcccgttttgactttttcataaggctatcaatgtagattttaaagtactcattctcactgagttgggcaagtttctggttgtcatcatatttactcaatataagtcgtaaatgctgatatgtatcaggcaaaatatcaagtatatatggtgggctatttttcaactgaagtttgggattttggcacagtcttaccactttgtccatgagcttccaagtcttctccacggtcctgcgatctgcggcagcttgcttagggggtccaactgcatcctgaatagcatcaataatacccaaaattcgaccttttcggggatttcctcctcgaccaccagggtttctgccattcattgagtttgccatctggaattttagttctttctttaaatcaacgcggtgagtcgttattcccaagaaccaaatgaaattaacacacaaatagcccatttgaaaagagaaaagagaaaaatgacaagagcggccacggaaaggaggagttcacttctctggctcctcgcctctgccctcaacccaaagctttgtttcaggacgcctgtgtcccttccctgctcaggccccttcccggcccctcgggtctgagctgcaggaggaaggtggactgggagggg

SEQ ID NO: 9419 - RNA, 5715 nt, Homo sapiens
  source 1..5715: mol_type = other RNA
aggaggcatcttgagaaatggaaggaatgtctaactttttggatcacagtgaaacaaagtctggatcacttccagacatcaacgagcagtcgcttttacaataaaaaaaaatttttttaggtttaatttcataggtgatagatagcaatgggtctttcttgacagtgtttaatagaaagttttcctcttttcattccattacgtatgaatttttgattcattctttttaaatgacaatactaatggttgctattgagtacaagatgcagagattttgctggaggctggtaaattttctctgcaaaacagatatccccccaccccccacccccaaatttcaggtccaggtttgctatatcatcactagtccttttttaattctcactggaaattttcaaatattgtttataaactgaatgagaatgtgctatgttctctaacattcttattttacatcattctctaatatattaggaatgttgcaacaatgttatcacaatgaagtggcaacttttggcctttagactgtacctatcatcagcaatcataaaaaggccaaaataaacagtgctattccaaggtgacatctgaaactgttaaaacaagtgaaaaatcataatgacaaaacaggggttcataaagcaaaagaaaatttgccaatgcaattttaaaagtgtaagaaacttcactcatgtacctactcatgggaagaacatctaaggcaaatgaaaaattcccctccagggacataaccagctcagaaccatctgaaaaaattcatacaaaagcagaaattacccaaggcctgtgagtcctcatctcataccatgaaagccagactgtcaaaaaaagggcacatgtcactttgcaaaggaatgtattaactcctctcccagggtcaacttagtctacgtgtcttttgtataacattaatttccaccagatctactagatgttcagtcatgtcctttcaggtcctgaaggcaggctcactctctgatgcatctttttatatcatggtgggtgtgaagtgaaaagaggagacacagaaatatgcacaaacccacaattagtccatatttagaaaactttctgtgggttcaagcatttacacagagatgattttatctcatttctccattaatttcccatttgaaatgaaaaccagctaattctaaattctaaagccctgggggaaaccttccaggctttgtctatcagacagactttgtcataaaaaacacagaaaaacaaaaataaaacattacgctggaatcagcttttgagagtttgtgctttaaaaacacagtgcctaacagcaccaagcatatcatagatgctcaataaatatttgtagatttattaagagtaataacatggtgtttaaagaaccaaccaccattttgtaaaataggcaaaactacattaatttctttcacctgatttgataaagcagtgtggagcaatgaatgagagaatctgcaaattaaatatgaactctaatttgattgcagagagaaaattactgagaactttgcaaaaaacattgccacagtagccttgacactcaacagtgcaacgaagagttaatgtttccactgcaatatgaactggttcccacagctcttaggagatagagtgtaatcacttaaatgggaaatgaactctaattccacttgagaaaaggtatgttatgttcataattttatctgaaaattattaatatatttcagggagatggtcctctcattcagcatccctcaaagtaatgcaggcataagtatcaggggaccttgttatataacttcagtacagcattgtcttatacaagtgttctctcttccacatctgtagtagctgctttctaatattgtagatttttacagttgtgacacccctgggatgacagacatgagaatatggaggattaaaggttacaaaacttaaacaaaaaagggaagctcctctatgttatgtgaaaaccccttacaaaaggcagtttattgacaaataaatgctttatacattcaggtttttcccatctctcaatagtgatggtttccaaagaagaaactcagtagtgaagaatacatacttttttttttttgcattagtttgatcagttgaaaatcagaaccttcaaagcatcttgtgaatgagagaaatggaactggacctgggcaaggcatggggatggtagagatccatatgaataaatgatttagctgttgatgtggacagcaagagagttggtgggaaatgttacagcagacctgaccacgctacaaagggtctgtgaagaacacagtacaggtatcaaaacaccaaaacaaaactaaactaaaaacaagaacaaactgcaactttgccaaactgtaaacaaggtaaagcatttcacaggttcaaagttcaagggaagtaaacgtctttaaattatttttgtcagttcaaccctgatttaaaaatatggctagcaaaaacaaggaagccacagctgtcgacatcctgagcaagcatcggtctcctttgagaagctgcactcccaagcctcttctcaagctgctacacgaggaggagacacttctctcttgaattccatctcagttctctttatttccacactcttggaatacatcgattgctttccattttggtgtctacagttctggctgctatagatttagacgtggggatactggaggagggaaggcaaattctcggaggatgctccgggcaacttcgacattattctgggctatctctaaggctctcttcacctcttcaaaggcataaccctctcccatgagttttgcaatttttgcatcgacattttccaatgccgcctcaggcccatggggttttctgtggtgaatttctggtgcagtcctgcgcggtcgtggtttagggggtctggctggtgcctgtgaaccatctgaacatgaaggaagctgatcatagtcctgtgatgttctgttagttttgacattttcacctggtaaccttctagcaggaggcaaaggaacttggccacttgctagatcaacaaagggatctgaaggaagaagaaaaagatcctgtcctgaggatggccggctactggagccaggaggttttgaatgttcaatgagactatgccttgcaggaggtgggggaggtgggagagatggagggagggcatcaaaagcatcttcacctaatggagggatgagaagatcataatcagagggcgtcctgttgagtgaagaaccatgctttggattgtcccgagttggaggcctggcaggtggtaatggcacgggatcagaggctgaatcaaaaacatctccctttaaatatatgcttaagtcagggatgtttgatttcttctctgaagatggaccatgtgttccattcagcatacagtgaccattatcacaagaccgaacaggaggttttacattatgacaatgagatggttgtgaattcagggaaacagggtgggatgaaggaatcttgtattcatcatcatcttcctctactgggtctcttgttttctctgaaagagaatttgctaacggaccagtacactttatgctagggaggagggtggtaactggaggaggaggagaaagccggggaggaacatcatattcttcacttccaaggtgaccattggaaaagaccttagctccttctaaaggcaaatcatggcgtctgtgtttccgcataagcactgggtcagagcccactctactgtgccttccattgacatttgaactcgctgtgattccaggttttggagagccctcccctaggagtcgacatcccacaagctgattagtcccaaacacatcccgagggcaccatgcttcaagaggcattggcgggtctctggaaggcacgctttccacatgatggatgtgtctactcagtctattgtctggtgggattggtggaggtctttcaggtggcggtggaggaggatctcttaagggaggaggtggtgctgggagtggtttatcttgttttctcaccatgcaaggagaagactttggtgaacccgttgggctgccacagggagatctaactatgcctttctgaattagatccaggcgaggaggcacgggtggcaggcttagatgtgggatctggagtgggtcaggctgtggctttcttctctgggcaaggggagaggatcctggtgatgtgactggtgagttctgcctgtcagtgcactttcggacgtttgccaaccgattcatcatcaaggactcctcacgatcatcatcgtcgtccaagtctagcatcggcatgccaaaggggtcaatgatgctgcaacacctggagccttcatctcttggatcaaaggggtccacgattatgggctcagttccttttatttcacaacgacagaaagggcagccctgaccatccgactcctgccatgccgtaaggcaagaggtgcacatcaaatgcccacaaggctcaatcttgacatctttgtcattctctgcacaaatcttacagagctgaaaagtggagcccatttcacaatataattcatattgttcctgtgtaacttttatatggtcatgaggtgtaggttcacataatccagttaaatcaggattataactcctcccatcaggataaagataaaatccttccctgctgccatcaatcagggcttgaaataagggcttgttatgaggtatggtctgtaagatattcccatccccagtcacatagccaatggcccactgtcccaatcgagtgcaacttaaccggaaaatatagcttccgggtttggtgctatatttctgtagtcgtgctttaacttcatcatatgtgagaaatgccatgtaacctggatgtgtcacagctaagaaattccaattccgcaaaatagagccccaaggctgaaacagcctggtaaaaatatcaaattcaaaaactgaaatgtaatcattgcaagttaaatcaattgttgattttagagccattgcttccaggccagagctaatctggtggacctcatgaaggcactgtctgaatactttccatggtacgatagttttgtctccaaaaaactttctccagaattcagcagcatctgcttttgtgatacgaaagttatctccctggaattgaccattgggaaagattgctttgatttctgccagcatgtgactgaagataagggacagttttgtgagatttcgtctgtcctgtgactgttcttcatacattctctccttgccttctttaaagagtcttattgcccgttttgactttttcataaggctatcaatgtagattttaaagtactcattctcactgagttgggcaagtttctggttgtcatcatatttactcaatataagtcgtaaatgctgatatgtatcaggcaaaatatcaagtatatatggtgggctatttttcaactgaagtttgggattttggcacagtcttaccactttgtccatgagcttccaagtcttctccacggtcctgcgatctgcggcagcttgcttagggggtccaactgcatcctgaatagcatcaataatacccaaaattcgaccttttcggggatttcctcctcgaccaccagggtttctgccattcattgagtttgccatctggaattttagttcaataaggggtggcaggtgggcgtgagcgtcgggaccgggagccaaagccatctggggctgaaaggcgggacttcctgct

SEQ ID NO: 9420 - RNA, 5736 nt, Homo sapiens
  source 1..5736: mol_type = other RNA
aggaggcatcttgagaaatggaaggaatgtctaactttttggatcacagtgaaacaaagtctggatcacttccagacatcaacgagcagtcgcttttacaataaaaaaaaatttttttaggtttaatttcataggtgatagatagcaatgggtctttcttgacagtgtttaatagaaagttttcctcttttcattccattacgtatgaatttttgattcattctttttaaatgacaatactaatggttgctattgagtacaagatgcagagattttgctggaggctggtaaattttctctgcaaaacagatatccccccaccccccacccccaaatttcaggtccaggtttgctatatcatcactagtccttttttaattctcactggaaattttcaaatattgtttataaactgaatgagaatgtgctatgttctctaacattcttattttacatcattctctaatatattaggaatgttgcaacaatgttatcacaatgaagtggcaacttttggcctttagactgtacctatcatcagcaatcataaaaaggccaaaataaacagtgctattccaaggtgacatctgaaactgttaaaacaagtgaaaaatcataatgacaaaacaggggttcataaagcaaaagaaaatttgccaatgcaattttaaaagtgtaagaaacttcactcatgtacctactcatgggaagaacatctaaggcaaatgaaaaattcccctccagggacataaccagctcagaaccatctgaaaaaattcatacaaaagcagaaattacccaaggcctgtgagtcctcatctcataccatgaaagccagactgtcaaaaaaagggcacatgtcactttgcaaaggaatgtattaactcctctcccagggtcaacttagtctacgtgtcttttgtataacattaatttccaccagatctactagatgttcagtcatgtcctttcaggtcctgaaggcaggctcactctctgatgcatctttttatatcatggtgggtgtgaagtgaaaagaggagacacagaaatatgcacaaacccacaattagtccatatttagaaaactttctgtgggttcaagcatttacacagagatgattttatctcatttctccattaatttcccatttgaaatgaaaaccagctaattctaaattctaaagccctgggggaaaccttccaggctttgtctatcagacagactttgtcataaaaaacacagaaaaacaaaaataaaacattacgctggaatcagcttttgagagtttgtgctttaaaaacacagtgcctaacagcaccaagcatatcatagatgctcaataaatatttgtagatttattaagagtaataacatggtgtttaaagaaccaaccaccattttgtaaaataggcaaaactacattaatttctttcacctgatttgataaagcagtgtggagcaatgaatgagagaatctgcaaattaaatatgaactctaatttgattgcagagagaaaattactgagaactttgcaaaaaacattgccacagtagccttgacactcaacagtgcaacgaagagttaatgtttccactgcaatatgaactggttcccacagctcttaggagatagagtgtaatcacttaaatgggaaatgaactctaattccacttgagaaaaggtatgttatgttcataattttatctgaaaattattaatatatttcagggagatggtcctctcattcagcatccctcaaagtaatgcaggcataagtatcaggggaccttgttatataacttcagtacagcattgtcttatacaagtgttctctcttccacatctgtagtagctgctttctaatattgtagatttttacagttgtgacacccctgggatgacagacatgagaatatggaggattaaaggttacaaaacttaaacaaaaaagggaagctcctctatgttatgtgaaaaccccttacaaaaggcagtttattgacaaataaatgctttatacattcaggtttttcccatctctcaatagtgatggtttccaaagaagaaactcagtagtgaagaatacatacttttttttttttgcattagtttgatcagttgaaaatcagaaccttcaaagcatcttgtgaatgagagaaatggaactggacctgggcaaggcatggggatggtagagatccatatgaataaatgatttagctgttgatgtggacagcaagagagttggtgggaaatgttacagcagacctgaccacgctacaaagggtctgtgaagaacacagtacaggtatcaaaacaccaaaacaaaactaaactaaaaacaagaacaaactgcaactttgccaaactgtaaacaaggtaaagcatttcacaggttcaaagttcaagggaagtaaacgtctttaaattatttttgtcagttcaaccctgatttaaaaatatggctagcaaaaacaaggaagccacagctgtcgacatcctgagcaagcatcggtctcctttgagaagctgcactcccaagcctcttctcaagctgctacacgaggaggagacacttctctcttgaattccatctcagttctctttatttccacactcttggaatacatcgattgctttccattttggtgtctacagttctggctgctatagatttagacgtggggatactggaggagggaaggcaaattctcggaggatgctccgggcaacttcgacattattctgggctatctctaaggctctcttcacctcttcaaaggcataaccctctcccatgagttttgcaatttttgcatcgacattttccaatgccgcctcaggcccatggggttttctgtggtgaatttctggtgcagtcctgcgcggtcgtggtttagggggtctggctggtgcctgtgaaccatctgaacatgaaggaagctgatcatagtcctgtgatgttctgttagttttgacattttcacctggtaaccttctagcaggaggcaaaggaacttggccacttgctagatcaacaaagggatctgaaggaagaagaaaaagatcctgtcctgaggatggccggctactggagccaggaggttttgaatgttcaatgagactatgccttgcaggaggtgggggaggtgggagagatggagggagggcatcaaaagcatcttcacctaatggagggatgagaagatcataatcagagggcgtcctgttgagtgaagaaccatgctttggattgtcccgagttggaggcctggcaggtggtaatggcacgggatcagaggctgaatcaaaaacatctccctttaaatatatgcttaagtcagggatgtttgatttcttctctgaagatggaccatgtgttccattcagcatacagtgaccattatcacaagaccgaacaggaggttttacattatgacaatgagatggttgtgaattcagggaaacagggtgggatgaaggaatcttgtattcatcatcatcttcctctactgggtctcttgttttctctgaaagagaatttgctaacggaccagtacactttatgctagggaggagggtggtaactggaggaggaggagaaagccggggaggaacatcatattcttcacttccaaggtgaccattggaaaagaccttagctccttctaaaggcaaatcatggcgtctgtgtttccgcataagcactgggtcagagcccactctactgtgccttccattgacatttgaactcgctgtgattccaggttttggagagccctcccctaggagtcgacatcccacaagctgattagtcccaaacacatcccgagggcaccatgcttcaagaggcattggcgggtctctggaaggcacgctttccacatgatggatgtgtctactcagtctattgtctggtgggattggtggaggtctttcaggtggcggtggaggaggatctcttaagggaggaggtggtgctgggagtggtttatcttgttttctcaccatgcaaggagaagactttggtgaacccgttgggctgccacagggagatctaactatgcctttctgaattagatccaggcgaggaggcacgggtggcaggcttagatgtgggatctggagtgggtcaggctgtggctttcttctctgggcaaggggagaggatcctggtgatgtgactggtgagttctgcctgtcagtgcactttcggacgtttgccaaccgattcatcatcaaggactcctcacgatcatcatcgtcgtccaagtctagcatcggcatgccaaaggggtcaatgatgctgcaacacctggagccttcatctcttggatcaaaggggtccacgattatgggctcagttccttttatttcacaacgacagaaagggcagccctgaccatccgactcctgccatgccgtaaggcaagaggtgcacatcaaatgcccacaaggctcaatcttgacatctttgtcattctctgcacaaatcttacagagctgaaaagtggagcccatttcacaatataattcatattgttcctgtgtaacttttatatggtcatgaggtgtaggttcacataatccagttaaatcaggattataactcctcccatcaggataaagataaaatccttccctgctgccatcaatcagggcttgaaataagggcttgttatgaggtatggtctgtaagatattcccatccccagtcacatagccaatggcccactgtcccaatcgagtgcaacttaaccggaaaatatagcttccgggtttggtgctatatttctgtagtcgtgctttaacttcatcatatgtgagaaatgccatgtaacctggatgtgtcacagctaagaaattccaattccgcaaaatagagccccaaggctgaaacagcctggtaaaaatatcaaattcaaaaactgaaatgtaatcattgcaagttaaatcaattgttgattttagagccattgcttccaggccagagctaatctggtggacctcatgaaggcactgtctgaatactttccatggtacgatagttttgtctccaaaaaactttctccagaattcagcagcatctgcttttgtgatacgaaagttatctccctggaattgaccattgggaaagattgctttgatttctgccagcatgtgactgaagataagggacagttttgtgagatttcgtctgtcctgtgactgttcttcatacattctctccttgccttctttaaagagtcttattgcccgttttgactttttcataaggctatcaatgtagattttaaagtactcattctcactgagttgggcaagtttctggttgtcatcatatttactcaatataagtcgtaaatgctgatatgtatcaggcaaaatatcaagtatatatggtgggctatttttcaactgaagtttgggattttggcacagtcttaccactttgtccatgagcttccaagtcttctccacggtcctgcgatctgcggcagcttgcttagggggtccaactgcatcctgaatagcatcaataatacccaaaattcgaccttttcggggatttcctcctcgaccaccagggtttctgccattcattgagtttgccatctggaattttagttcgtcaagacaaatccacacccgctctcccctcccgcccgactcggggaggccgcgggacgccgcagcagcactagcaggaggaggagaccgctcgctggac

SEQ ID NO: 9421 - RNA, 5763 nt, Homo sapiens
  source 1..5763: mol_type = other RNA
aggaggcatcttgagaaatggaaggaatgtctaactttttggatcacagtgaaacaaagtctggatcacttccagacatcaacgagcagtcgcttttacaataaaaaaaaatttttttaggtttaatttcataggtgatagatagcaatgggtctttcttgacagtgtttaatagaaagttttcctcttttcattccattacgtatgaatttttgattcattctttttaaatgacaatactaatggttgctattgagtacaagatgcagagattttgctggaggctggtaaattttctctgcaaaacagatatccccccaccccccacccccaaatttcaggtccaggtttgctatatcatcactagtccttttttaattctcactggaaattttcaaatattgtttataaactgaatgagaatgtgctatgttctctaacattcttattttacatcattctctaatatattaggaatgttgcaacaatgttatcacaatgaagtggcaacttttggcctttagactgtacctatcatcagcaatcataaaaaggccaaaataaacagtgctattccaaggtgacatctgaaactgttaaaacaagtgaaaaatcataatgacaaaacaggggttcataaagcaaaagaaaatttgccaatgcaattttaaaagtgtaagaaacttcactcatgtacctactcatgggaagaacatctaaggcaaatgaaaaattcccctccagggacataaccagctcagaaccatctgaaaaaattcatacaaaagcagaaattacccaaggcctgtgagtcctcatctcataccatgaaagccagactgtcaaaaaaagggcacatgtcactttgcaaaggaatgtattaactcctctcccagggtcaacttagtctacgtgtcttttgtataacattaatttccaccagatctactagatgttcagtcatgtcctttcaggtcctgaaggcaggctcactctctgatgcatctttttatatcatggtgggtgtgaagtgaaaagaggagacacagaaatatgcacaaacccacaattagtccatatttagaaaactttctgtgggttcaagcatttacacagagatgattttatctcatttctccattaatttcccatttgaaatgaaaaccagctaattctaaattctaaagccctgggggaaaccttccaggctttgtctatcagacagactttgtcataaaaaacacagaaaaacaaaaataaaacattacgctggaatcagcttttgagagtttgtgctttaaaaacacagtgcctaacagcaccaagcatatcatagatgctcaataaatatttgtagatttattaagagtaataacatggtgtttaaagaaccaaccaccattttgtaaaataggcaaaactacattaatttctttcacctgatttgataaagcagtgtggagcaatgaatgagagaatctgcaaattaaatatgaactctaatttgattgcagagagaaaattactgagaactttgcaaaaaacattgccacagtagccttgacactcaacagtgcaacgaagagttaatgtttccactgcaatatgaactggttcccacagctcttaggagatagagtgtaatcacttaaatgggaaatgaactctaattccacttgagaaaaggtatgttatgttcataattttatctgaaaattattaatatatttcagggagatggtcctctcattcagcatccctcaaagtaatgcaggcataagtatcaggggaccttgttatataacttcagtacagcattgtcttatacaagtgttctctcttccacatctgtagtagctgctttctaatattgtagatttttacagttgtgacacccctgggatgacagacatgagaatatggaggattaaaggttacaaaacttaaacaaaaaagggaagctcctctatgttatgtgaaaaccccttacaaaaggcagtttattgacaaataaatgctttatacattcaggtttttcccatctctcaatagtgatggtttccaaagaagaaactcagtagtgaagaatacatacttttttttttttgcattagtttgatcagttgaaaatcagaaccttcaaagcatcttgtgaatgagagaaatggaactggacctgggcaaggcatggggatggtagagatccatatgaataaatgatttagctgttgatgtggacagcaagagagttggtgggaaatgttacagcagacctgaccacgctacaaagggtctgtgaagaacacagtacaggtatcaaaacaccaaaacaaaactaaactaaaaacaagaacaaactgcaactttgccaaactgtaaacaaggtaaagcatttcacaggttcaaagttcaagggaagtaaacgtctttaaattatttttgtcagttcaaccctgatttaaaaatatggctagcaaaaacaaggaagccacagctgtcgacatcctgagcaagcatcggtctcctttgagaagctgcactcccaagcctcttctcaagctgctacacgaggaggagacacttctctcttgaattccatctcagttctctttatttccacactcttggaatacatcgattgctttccattttggtgtctacagttctggctgctatagatttagacgtggggatactggaggagggaaggcaaattctcggaggatgctccgggcaacttcgacattattctgggctatctctaaggctctcttcacctcttcaaaggcataaccctctcccatgagttttgcaatttttgcatcgacattttccaatgccgcctcaggcccatggggttttctgtggtgaatttctggtgcagtcctgcgcggtcgtggtttagggggtctggctggtgcctgtgaaccatctgaacatgaaggaagctgatcatagtcctgtgatgttctgttagttttgacattttcacctggtaaccttctagcaggaggcaaaggaacttggccacttgctagatcaacaaagggatctgaaggaagaagaaaaagatcctgtcctgaggatggccggctactggagccaggaggttttgaatgttcaatgagactatgccttgcaggaggtgggggaggtgggagagatggagggagggcatcaaaagcatcttcacctaatggagggatgagaagatcataatcagagggcgtcctgttgagtgaagaaccatgctttggattgtcccgagttggaggcctggcaggtggtaatggcacgggatcagaggctgaatcaaaaacatctccctttaaatatatgcttaagtcagggatgtttgatttcttctctgaagatggaccatgtgttccattcagcatacagtgaccattatcacaagaccgaacaggaggttttacattatgacaatgagatggttgtgaattcagggaaacagggtgggatgaaggaatcttgtattcatcatcatcttcctctactgggtctcttgttttctctgaaagagaatttgctaacggaccagtacactttatgctagggaggagggtggtaactggaggaggaggagaaagccggggaggaacatcatattcttcacttccaaggtgaccattggaaaagaccttagctccttctaaaggcaaatcatggcgtctgtgtttccgcataagcactgggtcagagcccactctactgtgccttccattgacatttgaactcgctgtgattccaggttttggagagccctcccctaggagtcgacatcccacaagctgattagtcccaaacacatcccgagggcaccatgcttcaagaggcattggcgggtctctggaaggcacgctttccacatgatggatgtgtctactcagtctattgtctggtgggattggtggaggtctttcaggtggcggtggaggaggatctcttaagggaggaggtggtgctgggagtggtttatcttgttttctcaccatgcaaggagaagactttggtgaacccgttgggctgccacagggagatctaactatgcctttctgaattagatccaggcgaggaggcacgggtggcaggcttagatgtgggatctggagtgggtcaggctgtggctttcttctctgggcaaggggagaggatcctggtgatgtgactggtgagttctgcctgtcagtgcactttcggacgtttgccaaccgattcatcatcaaggactcctcacgatcatcatcgtcgtccaagtctagcatcggcatgccaaaggggtcaatgatgctgcaacacctggagccttcatctcttggatcaaaggggtccacgattatgggctcagttccttttatttcacaacgacagaaagggcagccctgaccatccgactcctgccatgccgtaaggcaagaggtgcacatcaaatgcccacaaggctcaatcttgacatctttgtcattctctgcacaaatcttacagagctgaaaagtggagcccatttcacaatataattcatattgttcctgtgtaacttttatatggtcatgaggtgtaggttcacataatccagttaaatcaggattataactcctcccatcaggataaagataaaatccttccctgctgccatcaatcagggcttgaaataagggcttgttatgaggtatggtctgtaagatattcccatccccagtcacatagccaatggcccactgtcccaatcgagtgcaacttaaccggaaaatatagcttccgggtttggtgctatatttctgtagtcgtgctttaacttcatcatatgtgagaaatgccatgtaacctggatgtgtcacagctaagaaattccaattccgcaaaatagagccccaaggctgaaacagcctggtaaaaatatcaaattcaaaaactgaaatgtaatcattgcaagttaaatcaattgttgattttagagccattgcttccaggccagagctaatctggtggacctcatgaaggcactgtctgaatactttccatggtacgatagttttgtctccaaaaaactttctccagaattcagcagcatctgcttttgtgatacgaaagttatctccctggaattgaccattgggaaagattgctttgatttctgccagcatgtgactgaagataagggacagttttgtgagatttcgtctgtcctgtgactgttcttcatacattctctccttgccttctttaaagagtcttattgcccgttttgactttttcataaggctatcaatgtagattttaaagtactcattctcactgagttgggcaagtttctggttgtcatcatatttactcaatataagtcgtaaatgctgatatgtatcaggcaaaatatcaagtatatatggtgggctatttttcaactgaagtttgggattttggcacagtcttaccactttgtccatgagcttccaagtcttctccacggtcctgcgatctgcggcagcttgcttagggggtccaactgcatcctgaatagcatcaataatacccaaaattcgaccttttcggggatttcctcctcgaccaccagggtttctgccattcattgagtttgccatctggaattttagttcttcctagtcttttgtttcatagcaacagagtagtggctggaagggtgttgcttctccgctctgggcgggtccaacgctggagaaattcatctccctagggctgccaaacccttctacccaggacagc

SEQ ID NO: 9422 - RNA, 5912 nt, Homo sapiens
  source 1..5912: mol_type = other RNA
aggaggcatcttgagaaatggaaggaatgtctaactttttggatcacagtgaaacaaagtctggatcacttccagacatcaacgagcagtcgcttttacaataaaaaaaaatttttttaggtttaatttcataggtgatagatagcaatgggtctttcttgacagtgtttaatagaaagttttcctcttttcattccattacgtatgaatttttgattcattctttttaaatgacaatactaatggttgctattgagtacaagatgcagagattttgctggaggctggtaaattttctctgcaaaacagatatccccccaccccccacccccaaatttcaggtccaggtttgctatatcatcactagtccttttttaattctcactggaaattttcaaatattgtttataaactgaatgagaatgtgctatgttctctaacattcttattttacatcattctctaatatattaggaatgttgcaacaatgttatcacaatgaagtggcaacttttggcctttagactgtacctatcatcagcaatcataaaaaggccaaaataaacagtgctattccaaggtgacatctgaaactgttaaaacaagtgaaaaatcataatgacaaaacaggggttcataaagcaaaagaaaatttgccaatgcaattttaaaagtgtaagaaacttcactcatgtacctactcatgggaagaacatctaaggcaaatgaaaaattcccctccagggacataaccagctcagaaccatctgaaaaaattcatacaaaagcagaaattacccaaggcctgtgagtcctcatctcataccatgaaagccagactgtcaaaaaaagggcacatgtcactttgcaaaggaatgtattaactcctctcccagggtcaacttagtctacgtgtcttttgtataacattaatttccaccagatctactagatgttcagtcatgtcctttcaggtcctgaaggcaggctcactctctgatgcatctttttatatcatggtgggtgtgaagtgaaaagaggagacacagaaatatgcacaaacccacaattagtccatatttagaaaactttctgtgggttcaagcatttacacagagatgattttatctcatttctccattaatttcccatttgaaatgaaaaccagctaattctaaattctaaagccctgggggaaaccttccaggctttgtctatcagacagactttgtcataaaaaacacagaaaaacaaaaataaaacattacgctggaatcagcttttgagagtttgtgctttaaaaacacagtgcctaacagcaccaagcatatcatagatgctcaataaatatttgtagatttattaagagtaataacatggtgtttaaagaaccaaccaccattttgtaaaataggcaaaactacattaatttctttcacctgatttgataaagcagtgtggagcaatgaatgagagaatctgcaaattaaatatgaactctaatttgattgcagagagaaaattactgagaactttgcaaaaaacattgccacagtagccttgacactcaacagtgcaacgaagagttaatgtttccactgcaatatgaactggttcccacagctcttaggagatagagtgtaatcacttaaatgggaaatgaactctaattccacttgagaaaaggtatgttatgttcataattttatctgaaaattattaatatatttcagggagatggtcctctcattcagcatccctcaaagtaatgcaggcataagtatcaggggaccttgttatataacttcagtacagcattgtcttatacaagtgttctctcttccacatctgtagtagctgctttctaatattgtagatttttacagttgtgacacccctgggatgacagacatgagaatatggaggattaaaggttacaaaacttaaacaaaaaagggaagctcctctatgttatgtgaaaaccccttacaaaaggcagtttattgacaaataaatgctttatacattcaggtttttcccatctctcaatagtgatggtttccaaagaagaaactcagtagtgaagaatacatacttttttttttttgcattagtttgatcagttgaaaatcagaaccttcaaagcatcttgtgaatgagagaaatggaactggacctgggcaaggcatggggatggtagagatccatatgaataaatgatttagctgttgatgtggacagcaagagagttggtgggaaatgttacagcagacctgaccacgctacaaagggtctgtgaagaacacagtacaggtatcaaaacaccaaaacaaaactaaactaaaaacaagaacaaactgcaactttgccaaactgtaaacaaggtaaagcatttcacaggttcaaagttcaagggaagtaaacgtctttaaattatttttgtcagttcaaccctgatttaaaaatatggctagcaaaaacaaggaagccacagctgtcgacatcctgagcaagcatcggtctcctttgagaagctgcactcccaagcctcttctcaagctgctacacgaggaggagacacttctctcttgaattccatctcagttctctttatttccacactcttggaatacatcgattgctttccattttggtgtctacagttctggctgctatagatttagacgtggggatactggaggagggaaggcaaattctcggaggatgctccgggcaacttcgacattattctgggctatctctaaggctctcttcacctcttcaaaggcataaccctctcccatgagttttgcaatttttgcatcgacattttccaatgccgcctcaggcccatggggttttctgtggtgaatttctggtgcagtcctgcgcggtcgtggtttagggggtctggctggtgcctgtgaaccatctgaacatgaaggaagctgatcatagtcctgtgatgttctgttagttttgacattttcacctggtaaccttctagcaggaggcaaaggaacttggccacttgctagatcaacaaagggatctgaaggaagaagaaaaagatcctgtcctgaggatggccggctactggagccaggaggttttgaatgttcaatgagactatgccttgcaggaggtgggggaggtgggagagatggagggagggcatcaaaagcatcttcacctaatggagggatgagaagatcataatcagagggcgtcctgttgagtgaagaaccatgctttggattgtcccgagttggaggcctggcaggtggtaatggcacgggatcagaggctgaatcaaaaacatctccctttaaatatatgcttaagtcagggatgtttgatttcttctctgaagatggaccatgtgttccattcagcatacagtgaccattatcacaagaccgaacaggaggttttacattatgacaatgagatggttgtgaattcagggaaacagggtgggatgaaggaatcttgtattcatcatcatcttcctctactgggtctcttgttttctctgaaagagaatttgctaacggaccagtacactttatgctagggaggagggtggtaactggaggaggaggagaaagccggggaggaacatcatattcttcacttccaaggtgaccattggaaaagaccttagctccttctaaaggcaaatcatggcgtctgtgtttccgcataagcactgggtcagagcccactctactgtgccttccattgacatttgaactcgctgtgattccaggttttggagagccctcccctaggagtcgacatcccacaagctgattagtcccaaacacatcccgagggcaccatgcttcaagaggcattggcgggtctctggaaggcacgctttccacatgatggatgtgtctactcagtctattgtctggtgggattggtggaggtctttcaggtggcggtggaggaggatctcttaagggaggaggtggtgctgggagtggtttatcttgttttctcaccatgcaaggagaagactttggtgaacccgttgggctgccacagggagatctaactatgcctttctgaattagatccaggcgaggaggcacgggtggcaggcttagatgtgggatctggagtgggtcaggctgtggctttcttctctgggcaaggggagaggatcctggtgatgtgactggtgagttctgcctgtcagtgcactttcggacgtttgccaaccgattcatcatcaaggactcctcacgatcatcatcgtcgtccaagtctagcatcggcatgccaaaggggtcaatgatgctgcaacacctggagccttcatctcttggatcaaaggggtccacgattatgggctcagttccttttatttcacaacgacagaaagggcagccctgaccatccgactcctgccatgccgtaaggcaagaggtgcacatcaaatgcccacaaggctcaatcttgacatctttgtcattctctgcacaaatcttacagagctgaaaagtggagcccatttcacaatataattcatattgttcctgtgtaacttttatatggtcatgaggtgtaggttcacataatccagttaaatcaggattataactcctcccatcaggataaagataaaatccttccctgctgccatcaatcagggcttgaaataagggcttgttatgaggtatggtctgtaagatattcccatccccagtcacatagccaatggcccactgtcccaatcgagtgcaacttaaccggaaaatatagcttccgggtttggtgctatatttctgtagtcgtgctttaacttcatcatatgtgagaaatgccatgtaacctggatgtgtcacagctaagaaattccaattccgcaaaatagagccccaaggctgaaacagcctggtaaaaatatcaaattcaaaaactgaaatgtaatcattgcaagttaaatcaattgttgattttagagccattgcttccaggccagagctaatctggtggacctcatgaaggcactgtctgaatactttccatggtacgatagttttgtctccaaaaaactttctccagaattcagcagcatctgcttttgtgatacgaaagttatctccctggaattgaccattgggaaagattgctttgatttctgccagcatgtgactgaagataagggacagttttgtgagatttcgtctgtcctgtgactgttcttcatacattctctccttgccttctttaaagagtcttattgcccgttttgactttttcataaggctatcaatgtagattttaaagtactcattctcactgagttgggcaagtttctggttgtcatcatatttactcaatataagtcgtaaatgctgatatgtatcaggcaaaatatcaagtatatatggtgggctatttttcaactgaagtttgggattttggcacagtcttaccactttgtccatgagcttccaagtcttctccacggtcctgcgatctgcggcagcttgcttagggggtccaactgcatcctgaatagcatcaataatacccaaaattcgaccttttcggggatttcctcctcgaccaccagggtttctgccattcattgagtttgccatctggaattttagttctttcggcgccgtagctgtccagagacacgcgtgtgcgcgggtcccactccacacgcacgcagcccagtgtgtgtggggagccccggctgggagtgggatcgctgagaacagctcgctcccgaagaaggagcaacccagcgcgcaggcctccgagacgtggaaacgcaacaattaccgtcaagacaaatccacacccgctctcccctcccgcccgactcggggaggccgcgggacgccgcagcagcactagcaggaggaggagaccgctcgctggac

SEQ ID NO: 9423 - RNA, 5848 nt, Homo sapiens
  source 1..5848: mol_type = other RNA
aggaggcatcttgagaaatggaaggaatgtctaactttttggatcacagtgaaacaaagtctggatcacttccagacatcaacgagcagtcgcttttacaataaaaaaaaatttttttaggtttaatttcataggtgatagatagcaatgggtctttcttgacagtgtttaatagaaagttttcctcttttcattccattacgtatgaatttttgattcattctttttaaatgacaatactaatggttgctattgagtacaagatgcagagattttgctggaggctggtaaattttctctgcaaaacagatatccccccaccccccacccccaaatttcaggtccaggtttgctatatcatcactagtccttttttaattctcactggaaattttcaaatattgtttataaactgaatgagaatgtgctatgttctctaacattcttattttacatcattctctaatatattaggaatgttgcaacaatgttatcacaatgaagtggcaacttttggcctttagactgtacctatcatcagcaatcataaaaaggccaaaataaacagtgctattccaaggtgacatctgaaactgttaaaacaagtgaaaaatcataatgacaaaacaggggttcataaagcaaaagaaaatttgccaatgcaattttaaaagtgtaagaaacttcactcatgtacctactcatgggaagaacatctaaggcaaatgaaaaattcccctccagggacataaccagctcagaaccatctgaaaaaattcatacaaaagcagaaattacccaaggcctgtgagtcctcatctcataccatgaaagccagactgtcaaaaaaagggcacatgtcactttgcaaaggaatgtattaactcctctcccagggtcaacttagtctacgtgtcttttgtataacattaatttccaccagatctactagatgttcagtcatgtcctttcaggtcctgaaggcaggctcactctctgatgcatctttttatatcatggtgggtgtgaagtgaaaagaggagacacagaaatatgcacaaacccacaattagtccatatttagaaaactttctgtgggttcaagcatttacacagagatgattttatctcatttctccattaatttcccatttgaaatgaaaaccagctaattctaaattctaaagccctgggggaaaccttccaggctttgtctatcagacagactttgtcataaaaaacacagaaaaacaaaaataaaacattacgctggaatcagcttttgagagtttgtgctttaaaaacacagtgcctaacagcaccaagcatatcatagatgctcaataaatatttgtagatttattaagagtaataacatggtgtttaaagaaccaaccaccattttgtaaaataggcaaaactacattaatttctttcacctgatttgataaagcagtgtggagcaatgaatgagagaatctgcaaattaaatatgaactctaatttgattgcagagagaaaattactgagaactttgcaaaaaacattgccacagtagccttgacactcaacagtgcaacgaagagttaatgtttccactgcaatatgaactggttcccacagctcttaggagatagagtgtaatcacttaaatgggaaatgaactctaattccacttgagaaaaggtatgttatgttcataattttatctgaaaattattaatatatttcagggagatggtcctctcattcagcatccctcaaagtaatgcaggcataagtatcaggggaccttgttatataacttcagtacagcattgtcttatacaagtgttctctcttccacatctgtagtagctgctttctaatattgtagatttttacagttgtgacacccctgggatgacagacatgagaatatggaggattaaaggttacaaaacttaaacaaaaaagggaagctcctctatgttatgtgaaaaccccttacaaaaggcagtttattgacaaataaatgctttatacattcaggtttttcccatctctcaatagtgatggtttccaaagaagaaactcagtagtgaagaatacatacttttttttttttgcattagtttgatcagttgaaaatcagaaccttcaaagcatcttgtgaatgagagaaatggaactggacctgggcaaggcatggggatggtagagatccatatgaataaatgatttagctgttgatgtggacagcaagagagttggtgggaaatgttacagcagacctgaccacgctacaaagggtctgtgaagaacacagtacaggtatcaaaacaccaaaacaaaactaaactaaaaacaagaacaaactgcaactttgccaaactgtaaacaaggtaaagcatttcacaggttcaaagttcaagggaagtaaacgtctttaaattatttttgtcagttcaaccctgatttaaaaatatggctagcaaaaacaaggaagccacagctgtcgacatcctgagcaagcatcggtctcctttgagaagctgcactcccaagcctcttctcaagctgctacacgaggaggagacacttctctcttgaattccatctcagttctctttatttccacactcttggaatacatcgattgctttccattttggtgtctacagttctggctgctatagatttagacgtggggatactggaggagggaaggcaaattctcggaggatgctccgggcaacttcgacattattctgggctatctctaaggctctcttcacctcttcaaaggcataaccctctcccatgagttttgcaatttttgcatcgacattttccaatgccgcctcaggcccatggggttttctgtggtgaatttctggtgcagtcctgcgcggtcgtggtttagggggtctggctggtgcctgtgaaccatctgaacatgaaggaagctgatcatagtcctgtgatgttctgttagttttgacattttcacctggtaaccttctagcaggaggcaaaggaacttggccacttgctagatcaacaaagggatctgaaggaagaagaaaaagatcctgtcctgaggatggccggctactggagccaggaggttttgaatgttcaatgagactatgccttgcaggaggtgggggaggtgggagagatggagggagggcatcaaaagcatcttcacctaatggagggatgagaagatcataatcagagggcgtcctgttgagtgaagaaccatgctttggattgtcccgagttggaggcctggcaggtggtaatggcacgggatcagaggctgaatcaaaaacatctccctttaaatatatgcttaagtcagggatgtttgatttcttctctgaagatggaccatgtgttccattcagcatacagtgaccattatcacaagaccgaacaggaggttttacattatgacaatgagatggttgtgaattcagggaaacagggtgggatgaaggaatcttgtattcatcatcatcttcctctactgggtctcttgttttctctgaaagagaatttgctaacggaccagtacactttatgctagggaggagggtggtaactggaggaggaggagaaagccggggaggaacatcatattcttcacttccaaggtgaccattggaaaagaccttagctccttctaaaggcaaatcatggcgtctgtgtttccgcataagcactgggtcagagcccactctactgtgccttccattgacatttgaactcgctgtgattccaggttttggagagccctcccctaggagtcgacatcccacaagctgattagtcccaaacacatcccgagggcaccatgcttcaagaggcattggcgggtctctggaaggcacgctttccacatgatggatgtgtctactcagtctattgtctggtgggattggtggaggtctttcaggtggcggtggaggaggatctcttaagggaggaggtggtgctgggagtggtttatcttgttttctcaccatgcaaggagaagactttggtgaacccgttgggctgccacagggagatctaactatgcctttctgaattagatccaggcgaggaggcacgggtggcaggcttagatgtgggatctggagtgggtcaggctgtggctttcttctctgggcaaggggagaggatcctggtgatgtgactggtgagttctgcctgtcagtgcactttcggacgtttgccaaccgattcatcatcaaggactcctcacgatcatcatcgtcgtccaagtctagcatcggcatgccaaaggggtcaatgatgctgcaacacctggagccttcatctcttggatcaaaggggtccacgattatgggctcagttccttttatttcacaacgacagaaagggcagccctgaccatccgactcctgccatgccgtaaggcaagaggtgcacatcaaatgcccacaaggctcaatcttgacatctttgtcattctctgcacaaatcttacagagctgaaaagtggagcccatttcacaatataattcatattgttcctgtgtaacttttatatggtcatgaggtgtaggttcacataatccagttaaatcaggattataactcctcccatcaggataaagataaaatccttccctgctgccatcaatcagggcttgaaataagggcttgttatgaggtatggtctgtaagatattcccatccccagtcacatagccaatggcccactgtcccaatcgagtgcaacttaaccggaaaatatagcttccgggtttggtgctatatttctgtagtcgtgctttaacttcatcatatgtgagaaatgccatgtaacctggatgtgtcacagctaagaaattccaattccgcaaaatagagccccaaggctgaaacagcctggtaaaaatatcaaattcaaaaactgaaatgtaatcattgcaagttaaatcaattgttgattttagagccattgcttccaggccagagctaatctggtggacctcatgaaggcactgtctgaatactttccatggtacgatagttttgtctccaaaaaactttctccagaattcagcagcatctgcttttgtgatacgaaagttatctccctggaattgaccattgggaaagattgctttgatttctgccagcatgtgactgaagataagggacagttttgtgagatttcgtctgtcctgtgactgttcttcatacattctctccttgccttctttaaagagtcttattgcccgttttgactttttcataaggctatcaatgtagattttaaagtactcattctcactgagttgggcaagtttctggttgtcatcatatttactcaatataagtcgtaaatgctgatatgtatcaggcaaaatatcaagtatatatggtgggctatttttcaactgaagtttgggattttggcacagtcttaccactttgtccatgagcttccaagtcttctccacggtcctgcgatctgcggcagcttgcttagggggtccaactgcatcctgaatagcatcaataatacccaaaattcgaccttttcggggatttcctcctcgaccaccagggtttctgccattcattgagtttgccatctggaattttagttctttctttaaatcaacgcggtgagtcgttattcccaagaaccaaatgaaattaacacacaaatagcccatttgaaaagagaaaagagaaaaatgacaagagcggccacggaaaggaggagttcacttctctggctcctcgcctctgccctcaacccaaagctttgtttcaggacgcctgtgtcccttccctgctcaggccccttcccggcccc

SEQ ID NO: 9424 - RNA, 6056 nt, Homo sapiens
  source 1..6056: mol_type = other RNA
aggaggcatcttgagaaatggaaggaatgtctaactttttggatcacagtgaaacaaagtctggatcacttccagacatcaacgagcagtcgcttttacaataaaaaaaaatttttttaggtttaatttcataggtgatagatagcaatgggtctttcttgacagtgtttaatagaaagttttcctcttttcattccattacgtatgaatttttgattcattctttttaaatgacaatactaatggttgctattgagtacaagatgcagagattttgctggaggctggtaaattttctctgcaaaacagatatccccccaccccccacccccaaatttcaggtccaggtttgctatatcatcactagtccttttttaattctcactggaaattttcaaatattgtttataaactgaatgagaatgtgctatgttctctaacattcttattttacatcattctctaatatattaggaatgttgcaacaatgttatcacaatgaagtggcaacttttggcctttagactgtacctatcatcagcaatcataaaaaggccaaaataaacagtgctattccaaggtgacatctgaaactgttaaaacaagtgaaaaatcataatgacaaaacaggggttcataaagcaaaagaaaatttgccaatgcaattttaaaagtgtaagaaacttcactcatgtacctactcatgggaagaacatctaaggcaaatgaaaaattcccctccagggacataaccagctcagaaccatctgaaaaaattcatacaaaagcagaaattacccaaggcctgtgagtcctcatctcataccatgaaagccagactgtcaaaaaaagggcacatgtcactttgcaaaggaatgtattaactcctctcccagggtcaacttagtctacgtgtcttttgtataacattaatttccaccagatctactagatgttcagtcatgtcctttcaggtcctgaaggcaggctcactctctgatgcatctttttatatcatggtgggtgtgaagtgaaaagaggagacacagaaatatgcacaaacccacaattagtccatatttagaaaactttctgtgggttcaagcatttacacagagatgattttatctcatttctccattaatttcccatttgaaatgaaaaccagctaattctaaattctaaagccctgggggaaaccttccaggctttgtctatcagacagactttgtcataaaaaacacagaaaaacaaaaataaaacattacgctggaatcagcttttgagagtttgtgctttaaaaacacagtgcctaacagcaccaagcatatcatagatgctcaataaatatttgtagatttattaagagtaataacatggtgtttaaagaaccaaccaccattttgtaaaataggcaaaactacattaatttctttcacctgatttgataaagcagtgtggagcaatgaatgagagaatctgcaaattaaatatgaactctaatttgattgcagagagaaaattactgagaactttgcaaaaaacattgccacagtagccttgacactcaacagtgcaacgaagagttaatgtttccactgcaatatgaactggttcccacagctcttaggagatagagtgtaatcacttaaatgggaaatgaactctaattccacttgagaaaaggtatgttatgttcataattttatctgaaaattattaatatatttcagggagatggtcctctcattcagcatccctcaaagtaatgcaggcataagtatcaggggaccttgttatataacttcagtacagcattgtcttatacaagtgttctctcttccacatctgtagtagctgctttctaatattgtagatttttacagttgtgacacccctgggatgacagacatgagaatatggaggattaaaggttacaaaacttaaacaaaaaagggaagctcctctatgttatgtgaaaaccccttacaaaaggcagtttattgacaaataaatgctttatacattcaggtttttcccatctctcaatagtgatggtttccaaagaagaaactcagtagtgaagaatacatacttttttttttttgcattagtttgatcagttgaaaatcagaaccttcaaagcatcttgtgaatgagagaaatggaactggacctgggcaaggcatggggatggtagagatccatatgaataaatgatttagctgttgatgtggacagcaagagagttggtgggaaatgttacagcagacctgaccacgctacaaagggtctgtgaagaacacagtacaggtatcaaaacaccaaaacaaaactaaactaaaaacaagaacaaactgcaactttgccaaactgtaaacaaggtaaagcatttcacaggttcaaagttcaagggaagtaaacgtctttaaattatttttgtcagttcaaccctgatttaaaaatatggctagcaaaaacaaggaagccacagctgtcgacatcctgagcaagcatcggtctcctttgagaagctgcactcccaagcctcttctcaagctgctacacgaggaggagacacttctctcttgaattccatctcagttctctttatttccacactcttggaatacatcgattgctttccattttggtgtctacagttctggctgctatagatttagacgtggggatactggaggagggaaggcaaattctcggaggatgctccgggcaacttcgacattattctgggctatctctaaggctctcttcacctcttcaaaggcataaccctctcccatgagttttgcaatttttgcatcgacattttccaatgccgcctcaggcccatggggttttctgtggtgaatttctggtgcagtcctgcgcggtcgtggtttagggggtctggctggtgcctgtgaaccatctgaacatgaaggaagctgatcatagtcctgtgatgttctgttagttttgacattttcacctggtaaccttctagcaggaggcaaaggaacttggccacttgctagatcaacaaagggatctgaaggaagaagaaaaagatcctgtcctgaggatggccggctactggagccaggaggttttgaatgttcaatgagactatgccttgcaggaggtgggggaggtgggagagatggagggagggcatcaaaagcatcttcacctaatggagggatgagaagatcataatcagagggcgtcctgttgagtgaagaaccatgctttggattgtcccgagttggaggcctggcaggtggtaatggcacgggatcagaggctgaatcaaaaacatctccctttaaatatatgcttaagtcagggatgtttgatttcttctctgaagatggaccatgtgttccattcagcatacagtgaccattatcacaagaccgaacaggaggttttacattatgacaatgagatggttgtgaattcagggaaacagggtgggatgaaggaatcttgtattcatcatcatcttcctctactgggtctcttgttttctctgaaagagaatttgctaacggaccagtacactttatgctagggaggagggtggtaactggaggaggaggagaaagccggggaggaacatcatattcttcacttccaaggtgaccattggaaaagaccttagctccttctaaaggcaaatcatggcgtctgtgtttccgcataagcactgggtcagagcccactctactgtgccttccattgacatttgaactcgctgtgattccaggttttggagagccctcccctaggagtcgacatcccacaagctgattagtcccaaacacatcccgagggcaccatgcttcaagaggcattggcgggtctctggaaggcacgctttccacatgatggatgtgtctactcagtctattgtctggtgggattggtggaggtctttcaggtggcggtggaggaggatctcttaagggaggaggtggtgctgggagtggtttatcttgttttctcaccatgcaaggagaagactttggtgaacccgttgggctgccacagggagatctaactatgcctttctgaattagatccaggcgaggaggcacgggtggcaggcttagatgtgggatctggagtgggtcaggctgtggctttcttctctgggcaaggggagaggatcctggtgatgtgactggtgagttctgcctgtcagtgcactttcggacgtttgccaaccgattcatcatcaaggactcctcacgatcatcatcgtcgtccaagtctagcatcggcatgccaaaggggtcaatgatgctgcaacacctggagccttcatctcttggatcaaaggggtccacgattatgggctcagttccttttatttcacaacgacagaaagggcagccctgaccatccgactcctgccatgccgtaaggcaagaggtgcacatcaaatgcccacaaggctcaatcttgacatctttgtcattctctgcacaaatcttacagagctgaaaagtggagcccatttcacaatataattcatattgttcctgtgtaacttttatatggtcatgaggtgtaggttcacataatccagttaaatcaggattataactcctcccatcaggataaagataaaatccttccctgctgccatcaatcagggcttgaaataagggcttgttatgaggtatggtctgtaagatattcccatccccagtcacatagccaatggcccactgtcccaatcgagtgcaacttaaccggaaaatatagcttccgggtttggtgctatatttctgtagtcgtgctttaacttcatcatatgtgagaaatgccatgtaacctggatgtgtcacagctaagaaattccaattccgcaaaatagagccccaaggttcctagaatgagcagttaggtttaatgtaggaagattacttttactctcttccttgacaaggtgaagaagcaaagctcttactatttagaatgtctttgtatcatgttaaataaataagatattctgtaaaattatcagaaacctgaaacagcctggtaaaaatatcaaattcaaaaactgaaatgtaatcattgcaagttaaatcaattgttgattttagagccattgcttccaggccagagctaatctggtggacctcatgaaggcactgtctgaatactttccatggtacgatagttttgtctccaaaaaactttctccagaattcagcagcatctgcttttgtgatacgaaagttatctccctggaattgaccattgggaaagattgctttgatttctgccagcatgtgactgaagataagggacagttttgtgagatttcgtctgtcctgtgactgttcttcatacattctctccttgccttctttaaagagtcttattgcccgttttgactttttcataaggctatcaatgtagattttaaagtactcattctcactgagttgggcaagtttctggttgtcatcatatttactcaatataagtcgtaaatgctgatatgtatcaggcaaaatatcaagtatatatggtgggctatttttcaactgaagtttgggattttggcacagtcttaccactttgtccatgagcttccaagtcttctccacggtcctgcgatctgcggcagcttgcttagggggtccaactgcatcctgaatagcatcaataatacccaaaattcgaccttttcggggatttcctcctcgaccaccagggtttctgccattcattgagtttgccatctggaattttagttctttcggcgccgtagctgtccagagacacgcgtgtgcgcgggtcccactccacacgcacgcagcccagtgtgtgtggggagccccggctgggagtgggatcgctgagaacagctcgctcccgaagaaggagcaacccagcgcgcaggcctccgagacgtggaaacgcaacaattaccgtcaagacaaatccacacccgctctcccctcccgcccgactcggggaggccgcgggacgccgcagcagcactagcaggaggaggagaccgctcgctggac

SEQ ID NO: 9425 - RNA, 5579 nt, Homo sapiens
  source 1..5579: mol_type = other RNA
aggaggcatcttgagaaatggaaggaatgtctaactttttggatcacagtgaaacaaagtctggatcacttccagacatcaacgagcagtcgcttttacaataaaaaaaaatttttttaggtttaatttcataggtgatagatagcaatgggtctttcttgacagtgtttaatagaaagttttcctcttttcattccattacgtatgaatttttgattcattctttttaaatgacaatactaatggttgctattgagtacaagatgcagagattttgctggaggctggtaaattttctctgcaaaacagatatccccccaccccccacccccaaatttcaggtccaggtttgctatatcatcactagtccttttttaattctcactggaaattttcaaatattgtttataaactgaatgagaatgtgctatgttctctaacattcttattttacatcattctctaatatattaggaatgttgcaacaatgttatcacaatgaagtggcaacttttggcctttagactgtacctatcatcagcaatcataaaaaggccaaaataaacagtgctattccaaggtgacatctgaaactgttaaaacaagtgaaaaatcataatgacaaaacaggggttcataaagcaaaagaaaatttgccaatgcaattttaaaagtgtaagaaacttcactcatgtacctactcatgggaagaacatctaaggcaaatgaaaaattcccctccagggacataaccagctcagaaccatctgaaaaaattcatacaaaagcagaaattacccaaggcctgtgagtcctcatctcataccatgaaagccagactgtcaaaaaaagggcacatgtcactttgcaaaggaatgtattaactcctctcccagggtcaacttagtctacgtgtcttttgtataacattaatttccaccagatctactagatgttcagtcatgtcctttcaggtcctgaaggcaggctcactctctgatgcatctttttatatcatggtgggtgtgaagtgaaaagaggagacacagaaatatgcacaaacccacaattagtccatatttagaaaactttctgtgggttcaagcatttacacagagatgattttatctcatttctccattaatttcccatttgaaatgaaaaccagctaattctaaattctaaagccctgggggaaaccttccaggctttgtctatcagacagactttgtcataaaaaacacagaaaaacaaaaataaaacattacgctggaatcagcttttgagagtttgtgctttaaaaacacagtgcctaacagcaccaagcatatcatagatgctcaataaatatttgtagatttattaagagtaataacatggtgtttaaagaaccaaccaccattttgtaaaataggcaaaactacattaatttctttcacctgatttgataaagcagtgtggagcaatgaatgagagaatctgcaaattaaatatgaactctaatttgattgcagagagaaaattactgagaactttgcaaaaaacattgccacagtagccttgacactcaacagtgcaacgaagagttaatgtttccactgcaatatgaactggttcccacagctcttaggagatagagtgtaatcacttaaatgggaaatgaactctaattccacttgagaaaaggtatgttatgttcataattttatctgaaaattattaatatatttcagggagatggtcctctcattcagcatccctcaaagtaatgcaggcataagtatcaggggaccttgttatataacttcagtacagcattgtcttatacaagtgttctctcttccacatctgtagtagctgctttctaatattgtagatttttacagttgtgacacccctgggatgacagacatgagaatatggaggattaaaggttacaaaacttaaacaaaaaagggaagctcctctatgttatgtgaaaaccccttacaaaaggcagtttattgacaaataaatgctttatacattcaggtttttcccatctctcaatagtgatggtttccaaagaagaaactcagtagtgaagaatacatacttttttttttttgcattagtttgatcagttgaaaatcagaaccttcaaagcatcttgtgaatgagagaaatggaactggacctgggcaaggcatggggatggtagagatccatatgaataaatgatttagctgttgatgtggacagcaagagagttggtgggaaatgttacagcagacctgaccacgctacaaagggtctgtgaagaacacagtacaggtatcaaaacaccaaaacaaaactaaactaaaaacaagaacaaactgcaactttgccaaactgtaaacaaggtaaagcatttcacaggttcaaagttcaagggaagtaaacgtctttaaattatttttgtcagttcaaccctgatttaaaaatatggctagcaaaaacaaggaagccacagctgtcgacatcctgagcaagcatcggtctcctttgagaagctgcactcccaagcctcttctcaagctgctacacgaggaggagacacttctctcttgaattccatctcagttctctttatttccacactcttggaatacatcgattgctttccattttggtgtctacagttctggctgctatagatttagacgtggggatactggaggagggaaggcaaattctcggaggatgctccgggcaacttcgacattattctgggctatctctaaggctctcttcacctcttcaaaggcataaccctctcccatgagttttgcaatttttgcatcgacattttccaatgccgcctcaggcccatggggttttctgtggtgaatttctggtgcagtcctgcgcggtcgtggtttagggggtctggctggtgcctgtgaaccatctgaacatgaaggaagctgatcatagtcctgtgatgttctgttagttttgacattttcacctggtaaccttctagcaggaggcaaaggaacttggccacttgctagatcaacaaagggatctgaaggaagaagaaaaagatcctgtcctgaggatggccggctactggagccaggaggttttgaatgttcaatgagactatgccttgcaggaggtgggggaggtgggagagatggagggagggcatcaaaagcatcttcacctaatggagggatgagaagatcataatcagagggcgtcctgttgagtgaagaaccatgctttggattgtcccgagttggaggcctggcaggtggtaatggcacgggatcagaggctgaatcaaaaacatctccctttaaatatatgcttaagtcagggatgtttgatttcttctctgaagatggaccatgtgttccattcagcatacagtgaccattatcacaagaccgaacaggaggttttacattatgacaatgagatggttgtgaattcagggaaacagggtgggatgaaggaatcttgtattcatcatcatcttcctctactgggtctcttgttttctctgaaagagaatttgctaacggaccagtacactttatgctagggaggagggtggtaactggaggaggaggagaaagccggggaggaacatcatattcttcacttccaaggtgaccattggaaaagaccttagctccttctaaaggcaaatcatggcgtctgtgtttccgcataagcactgggtcagagcccactctactgtgccttccattgacatttgaactcgctgtgattccaggttttggagagccctcccctaggagtcgacatcccacaagctgattagtcccaaacacatcccgagggcaccatgcttcaagaggcattggcgggtctctggaaggcacgctttccacatgatggatgtgtctactcagtctattgtctggtgggattggtggaggtctttcaggtggcggtggaggaggatctcttaagggaggaggtggtgctgggagtggtttatcttgttttctcaccatgcaaggagaagactttggtgaacccgttgggctgccacagggagatctaactatgcctttctgaattagatccaggcgaggaggcacgggtggcaggcttagatgtgggatctggagtgggtcaggctgtggctttcttctctgggcaaggggagaggatcctggtgatgtgactggtgagttctgcctgtcagtgcactttcggacgtttgccaaccgattcatcatcaaggactcctcacgatcatcatcgtcgtccaagtctagcatcggcatgccaaaggggtcaatgatgctgcaacacctggagccttcatctcttggatcaaaggggtccacgattatgggctcagttccttttatttcacaacgacagaaagggcagccctgaccatccgactcctgccatgccgtaaggcaagaggtgcacatcaaatgcccacaaggctcaatcttgacatctttgtcattctctgcacaaatcttacagagctgaaaagtggagcccatttcacaatataattcatattgttcctgtgtaacttttatatggtcatgaggtgtaggttcacataatccagttaaatcaggattataactcctcccatcaggataaagataaaatccttccctgctgccatcaatcagggcttgaaataagggcttgttatgaggtatggtctgtaagatattcccatccccagtcacatagccaatggcccactgtcccaatcgagtgcaacttaaccggaaaatatagcttccgggtttggtgctatatttctgtagtcgtgctttaacttcatcatatgtgagaaatgccatgtaacctggatgtgtcacagctaagaaattccaattccgcaaaatagagccccaaggttgtctccaaaaaactttctccagaattcagcagcatctgcttttgtgatacgaaagttatctccctggaattgaccattgggaaagattgctttgatttctgccagcatgtgactgaagataagggacagttttgtgagatttcgtctgtcctgtgactgttcttcatacattctctccttgccttctttaaagagtcttattgcccgttttgactttttcataaggctatcaatgtagattttaaagtactcattctcactgagttgggcaagtttctggttgtcatcatatttactcaatataagtcgtaaatgctgatatgtatcaggcaaaatatcaagtatatatggtgggctatttttcaactgaagtttgggattttggcacagtcttaccactttgtccatgagcttccaagtcttctccacggtcctgcgatctgcggcagcttgcttagggggtccaactgcatcctgaatagcatcaataatacccaaaattcgaccttttcggggatttcctcctcgaccaccagggtttctgccattcattgagtttgccatctggaattttagttcgtcaagacaaatccacacccgctctcccctcccgcccgactcggggaggccgcgggacgccgcagcagcactagcaggaggaggagaccgctcgctggac

SEQ ID NO: 9426 - RNA, 5589 nt, Homo sapiens
  source 1..5589: mol_type = other RNA
aggaggcatcttgagaaatggaaggaatgtctaactttttggatcacagtgaaacaaagtctggatcacttccagacatcaacgagcagtcgcttttacaataaaaaaaaatttttttaggtttaatttcataggtgatagatagcaatgggtctttcttgacagtgtttaatagaaagttttcctcttttcattccattacgtatgaatttttgattcattctttttaaatgacaatactaatggttgctattgagtacaagatgcagagattttgctggaggctggtaaattttctctgcaaaacagatatccccccaccccccacccccaaatttcaggtccaggtttgctatatcatcactagtccttttttaattctcactggaaattttcaaatattgtttataaactgaatgagaatgtgctatgttctctaacattcttattttacatcattctctaatatattaggaatgttgcaacaatgttatcacaatgaagtggcaacttttggcctttagactgtacctatcatcagcaatcataaaaaggccaaaataaacagtgctattccaaggtgacatctgaaactgttaaaacaagtgaaaaatcataatgacaaaacaggggttcataaagcaaaagaaaatttgccaatgcaattttaaaagtgtaagaaacttcactcatgtacctactcatgggaagaacatctaaggcaaatgaaaaattcccctccagggacataaccagctcagaaccatctgaaaaaattcatacaaaagcagaaattacccaaggcctgtgagtcctcatctcataccatgaaagccagactgtcaaaaaaagggcacatgtcactttgcaaaggaatgtattaactcctctcccagggtcaacttagtctacgtgtcttttgtataacattaatttccaccagatctactagatgttcagtcatgtcctttcaggtcctgaaggcaggctcactctctgatgcatctttttatatcatggtgggtgtgaagtgaaaagaggagacacagaaatatgcacaaacccacaattagtccatatttagaaaactttctgtgggttcaagcatttacacagagatgattttatctcatttctccattaatttcccatttgaaatgaaaaccagctaattctaaattctaaagccctgggggaaaccttccaggctttgtctatcagacagactttgtcataaaaaacacagaaaaacaaaaataaaacattacgctggaatcagcttttgagagtttgtgctttaaaaacacagtgcctaacagcaccaagcatatcatagatgctcaataaatatttgtagatttattaagagtaataacatggtgtttaaagaaccaaccaccattttgtaaaataggcaaaactacattaatttctttcacctgatttgataaagcagtgtggagcaatgaatgagagaatctgcaaattaaatatgaactctaatttgattgcagagagaaaattactgagaactttgcaaaaaacattgccacagtagccttgacactcaacagtgcaacgaagagttaatgtttccactgcaatatgaactggttcccacagctcttaggagatagagtgtaatcacttaaatgggaaatgaactctaattccacttgagaaaaggtatgttatgttcataattttatctgaaaattattaatatatttcagggagatggtcctctcattcagcatccctcaaagtaatgcaggcataagtatcaggggaccttgttatataacttcagtacagcattgtcttatacaagtgttctctcttccacatctgtagtagctgctttctaatattgtagatttttacagttgtgacacccctgggatgacagacatgagaatatggaggattaaaggttacaaaacttaaacaaaaaagggaagctcctctatgttatgtgaaaaccccttacaaaaggcagtttattgacaaataaatgctttatacattcaggtttttcccatctctcaatagtgatggtttccaaagaagaaactcagtagtgaagaatacatacttttttttttttgcattagtttgatcagttgaaaatcagaaccttcaaagcatcttgtgaatgagagaaatggaactggacctgggcaaggcatggggatggtagagatccatatgaataaatgatttagctgttgatgtggacagcaagagagttggtgggaaatgttacagcagacctgaccacgctacaaagggtctgtgaagaacacagtacaggtatcaaaacaccaaaacaaaactaaactaaaaacaagaacaaactgcaactttgccaaactgtaaacaaggtaaagcatttcacaggttcaaagttcaagggaagtaaacgtctttaaattatttttgtcagttcaaccctgatttaaaaatatggctagcaaaaacaaggaagccacagctgtcgacatcctgagcaagcatcggtctcctttgagaagctgcactcccaagcctcttctcaagctgctacacgaggaggagacacttctctcttgaattccatctcagttctctttatttccacactcttggaatacatcgattgctttccattttggtgtctacagttctggctgctatagatttagacgtggggatactggaggagggaaggcaaattctcggaggatgctccgggcaacttcgacattattctgggctatctctaaggctctcttcacctcttcaaaggcataaccctctcccatgagttttgcaatttttgcatcgacattttccaatgccgcctcaggcccatggggttttctgtggtgaatttctggtgcagtcctgcgcggtcgtggtttagggggtctggctggtgcctgtgaaccatctgaacatgaaggaagctgatcatagtcctgtgatgttctgttagttttgacattttcacctggtaaccttctagcaggaggcaaaggaacttggccacttgctagatcaacaaagggatctgaaggaagaagaaaaagatcctgtcctgaggatggccggctactggagccaggaggttttgaatgttcaatgagactatgccttgcaggaggtgggggaggtgggagagatggagggagggcatcaaaagcatcttcacctaatggagggatgagaagatcataatcagagggcgtcctgttgagtgaagaaccatgctttggattgtcccgagttggaggcctggcaggtggtaatggcacgggatcagaggctgaatcaaaaacatctccctttaaatatatgcttaagtcagggatgtttgatttcttctctgaagatggaccatgtgttccattcagcatacagtgaccattatcacaagactttatgctagggaggagggtggtaactggaggaggaggagaaagccggggaggaacatcatattcttcacttccaaggtgaccattggaaaagaccttagctccttctaaaggcaaatcatggcgtctgtgtttccgcataagcactgggtcagagcccactctactgtgccttccattgacatttgaactcgctgtgattccaggttttggagagccctcccctaggagtcgacatcccacaagctgattagtcccaaacacatcccgagggcaccatgcttcaagaggcattggcgggtctctggaaggcacgctttccacatgatggatgtgtctactcagtctattgtctggtgggattggtggaggtctttcaggtggcggtggaggaggatctcttaagggaggaggtggtgctgggagtggtttatcttgttttctcaccatgcaaggagaagactttggtgaacccgttgggctgccacagggagatctaactatgcctttctgaattagatccaggcgaggaggcacgggtggcaggcttagatgtgggatctggagtgggtcaggctgtggctttcttctctgggcaaggggagaggatcctggtgatgtgactggtgagttctgcctgtcagtgcactttcggacgtttgccaaccgattcatcatcaaggactcctcacgatcatcatcgtcgtccaagtctagcatcggcatgccaaaggggtcaatgatgctgcaacacctggagccttcatctcttggatcaaaggggtccacgattatgggctcagttccttttatttcacaacgacagaaagggcagccctgaccatccgactcctgccatgccgtaaggcaagaggtgcacatcaaatgcccacaaggctcaatcttgacatctttgtcattctctgcacaaatcttacagagctgaaaagtggagcccatttcacaatataattcatattgttcctgtgtaacttttatatggtcatgaggtgtaggttcacataatccagttaaatcaggattataactcctcccatcaggataaagataaaatccttccctgctgccatcaatcagggcttgaaataagggcttgttatgaggtatggtctgtaagatattcccatccccagtcacatagccaatggcccactgtcccaatcgagtgcaacttaaccggaaaatatagcttccgggtttggtgctatatttctgtagtcgtgctttaacttcatcatatgtgagaaatgccatgtaacctggatgtgtcacagctaagaaattccaattccgcaaaatagagccccaaggctgaaacagcctggtaaaaatatcaaattcaaaaactgaaatgtaatcattgcaagttaaatcaattgttgattttagagccattgcttccaggccagagctaatctggtggacctcatgaaggcactgtctgaatactttccatggtacgatagttttgtctccaaaaaactttctccagaattcagcagcatctgcttttgtgatacgaaagttatctccctggaattgaccattgggaaagattgctttgatttctgccagcatgtgactgaagataagggacagttttgtgagatttcgtctgtcctgtgactgttcttcatacattctctccttgccttctttaaagagtcttattgcccgttttgactttttcataaggctatcaatgtagattttaaagtactcattctcactgagttgggcaagtttctggttgtcatcatatttactcaatataagtcgtaaatgctgatatgtatcaggcaaaatatcaagtatatatggtgggctatttttcaactgaagtttgggattttggcacagtcttaccactttgtccatgagcttccaagtcttctccacggtcctgcgatctgcggcagcttgcttagggggtccaactgcatcctgaatagcatcaataatacccaaaattcgaccttttcggggatttcctcctcgaccaccagggtttctgccattcattgagtttgccatctggaattttagttcgtcaagacaaatccacacccgctctcccctcccgcccgactcggggaggccgcgggacgccgcagcagcactagcaggaggaggagaccgctcgctggac

SEQ ID NO: 9427 - RNA, 5765 nt, Homo sapiens
  source 1..5765: mol_type = other RNA
aggaggcatcttgagaaatggaaggaatgtctaactttttggatcacagtgaaacaaagtctggatcacttccagacatcaacgagcagtcgcttttacaataaaaaaaaatttttttaggtttaatttcataggtgatagatagcaatgggtctttcttgacagtgtttaatagaaagttttcctcttttcattccattacgtatgaatttttgattcattctttttaaatgacaatactaatggttgctattgagtacaagatgcagagattttgctggaggctggtaaattttctctgcaaaacagatatccccccaccccccacccccaaatttcaggtccaggtttgctatatcatcactagtccttttttaattctcactggaaattttcaaatattgtttataaactgaatgagaatgtgctatgttctctaacattcttattttacatcattctctaatatattaggaatgttgcaacaatgttatcacaatgaagtggcaacttttggcctttagactgtacctatcatcagcaatcataaaaaggccaaaataaacagtgctattccaaggtgacatctgaaactgttaaaacaagtgaaaaatcataatgacaaaacaggggttcataaagcaaaagaaaatttgccaatgcaattttaaaagtgtaagaaacttcactcatgtacctactcatgggaagaacatctaaggcaaatgaaaaattcccctccagggacataaccagctcagaaccatctgaaaaaattcatacaaaagcagaaattacccaaggcctgtgagtcctcatctcataccatgaaagccagactgtcaaaaaaagggcacatgtcactttgcaaaggaatgtattaactcctctcccagggtcaacttagtctacgtgtcttttgtataacattaatttccaccagatctactagatgttcagtcatgtcctttcaggtcctgaaggcaggctcactctctgatgcatctttttatatcatggtgggtgtgaagtgaaaagaggagacacagaaatatgcacaaacccacaattagtccatatttagaaaactttctgtgggttcaagcatttacacagagatgattttatctcatttctccattaatttcccatttgaaatgaaaaccagctaattctaaattctaaagccctgggggaaaccttccaggctttgtctatcagacagactttgtcataaaaaacacagaaaaacaaaaataaaacattacgctggaatcagcttttgagagtttgtgctttaaaaacacagtgcctaacagcaccaagcatatcatagatgctcaataaatatttgtagatttattaagagtaataacatggtgtttaaagaaccaaccaccattttgtaaaataggcaaaactacattaatttctttcacctgatttgataaagcagtgtggagcaatgaatgagagaatctgcaaattaaatatgaactctaatttgattgcagagagaaaattactgagaactttgcaaaaaacattgccacagtagccttgacactcaacagtgcaacgaagagttaatgtttccactgcaatatgaactggttcccacagctcttaggagatagagtgtaatcacttaaatgggaaatgaactctaattccacttgagaaaaggtatgttatgttcataattttatctgaaaattattaatatatttcagggagatggtcctctcattcagcatccctcaaagtaatgcaggcataagtatcaggggaccttgttatataacttcagtacagcattgtcttatacaagtgttctctcttccacatctgtagtagctgctttctaatattgtagatttttacagttgtgacacccctgggatgacagacatgagaatatggaggattaaaggttacaaaacttaaacaaaaaagggaagctcctctatgttatgtgaaaaccccttacaaaaggcagtttattgacaaataaatgctttatacattcaggtttttcccatctctcaatagtgatggtttccaaagaagaaactcagtagtgaagaatacatacttttttttttttgcattagtttgatcagttgaaaatcagaaccttcaaagcatcttgtgaatgagagaaatggaactggacctgggcaaggcatggggatggtagagatccatatgaataaatgatttagctgttgatgtggacagcaagagagttggtgggaaatgttacagcagacctgaccacgctacaaagggtctgtgaagaacacagtacaggtatcaaaacaccaaaacaaaactaaactaaaaacaagaacaaactgcaactttgccaaactgtaaacaaggtaaagcatttcacaggttcaaagttcaagggaagtaaacgtctttaaattatttttgtcagttcaaccctgatttaaaaatatggctagcaaaaacaaggaagccacagctgtcgacatcctgagcaagcatcggtctcctttgagaagctgcactcccaagcctcttctcaagctgctacacgaggaggagacacttctctcttgaattccatctcagttctctttatttccacactcttggaatacatcgattgctttccattttggtgtctacagttctggctgctatagatttagacgtggggatactggaggagggaaggcaaattctcggaggatgctccgggcaacttcgacattattctgggctatctctaaggctctcttcacctcttcaaaggcataaccctctcccatgagttttgcaatttttgcatcgacattttccaatgccgcctcaggcccatggggttttctgtggtgaatttctggtgcagtcctgcgcggtcgtggtttagggggtctggctggtgcctgtgaaccatctgaacatgaaggaagctgatcatagtcctgtgatgttctgttagttttgacattttcacctggtaaccttctagcaggaggcaaaggaacttggccacttgctagatcaacaaagggatctgaaggaagaagaaaaagatcctgtcctgaggatggccggctactggagccaggaggttttgaatgttcaatgagactatgccttgcaggaggtgggggaggtgggagagatggagggagggcatcaaaagcatcttcacctaatggagggatgagaagatcataatcagagggcgtcctgttgagtgaagaaccatgctttggattgtcccgagttggaggcctggcaggtggtaatggcacgggatcagaggctgaatcaaaaacatctccctttaaatatatgcttaagtcagggatgtttgatttcttctctgaagatggaccatgtgttccattcagcatacagtgaccattatcacaagactttatgctagggaggagggtggtaactggaggaggaggagaaagccggggaggaacatcatattcttcacttccaaggtgaccattggaaaagaccttagctccttctaaaggcaaatcatggcgtctgtgtttccgcataagcactgggtcagagcccactctactgtgccttccattgacatttgaactcgctgtgattccaggttttggagagccctcccctaggagtcgacatcccacaagctgattagtcccaaacacatcccgagggcaccatgcttcaagaggcattggcgggtctctggaaggcacgctttccacatgatggatgtgtctactcagtctattgtctggtgggattggtggaggtctttcaggtggcggtggaggaggatctcttaagggaggaggtggtgctgggagtggtttatcttgttttctcaccatgcaaggagaagactttggtgaacccgttgggctgccacagggagatctaactatgcctttctgaattagatccaggcgaggaggcacgggtggcaggcttagatgtgggatctggagtgggtcaggctgtggctttcttctctgggcaaggggagaggatcctggtgatgtgactggtgagttctgcctgtcagtgcactttcggacgtttgccaaccgattcatcatcaaggactcctcacgatcatcatcgtcgtccaagtctagcatcggcatgccaaaggggtcaatgatgctgcaacacctggagccttcatctcttggatcaaaggggtccacgattatgggctcagttccttttatttcacaacgacagaaagggcagccctgaccatccgactcctgccatgccgtaaggcaagaggtgcacatcaaatgcccacaaggctcaatcttgacatctttgtcattctctgcacaaatcttacagagctgaaaagtggagcccatttcacaatataattcatattgttcctgtgtaacttttatatggtcatgaggtgtaggttcacataatccagttaaatcaggattataactcctcccatcaggataaagataaaatccttccctgctgccatcaatcagggcttgaaataagggcttgttatgaggtatggtctgtaagatattcccatccccagtcacatagccaatggcccactgtcccaatcgagtgcaacttaaccggaaaatatagcttccgggtttggtgctatatttctgtagtcgtgctttaacttcatcatatgtgagaaatgccatgtaacctggatgtgtcacagctaagaaattccaattccgcaaaatagagccccaaggctgaaacagcctggtaaaaatatcaaattcaaaaactgaaatgtaatcattgcaagttaaatcaattgttgattttagagccattgcttccaggccagagctaatctggtggacctcatgaaggcactgtctgaatactttccatggtacgatagttttgtctccaaaaaactttctccagaattcagcagcatctgcttttgtgatacgaaagttatctccctggaattgaccattgggaaagattgctttgatttctgccagcatgtgactgaagataagggacagttttgtgagatttcgtctgtcctgtgactgttcttcatacattctctccttgccttctttaaagagtcttattgcccgttttgactttttcataaggctatcaatgtagattttaaagtactcattctcactgagttgggcaagtttctggttgtcatcatatttactcaatataagtcgtaaatgctgatatgtatcaggcaaaatatcaagtatatatggtgggctatttttcaactgaagtttgggattttggcacagtcttaccactttgtccatgagcttccaagtcttctccacggtcctgcgatctgcggcagcttgcttagggggtccaactgcatcctgaatagcatcaataatacccaaaattcgaccttttcggggatttcctcctcgaccaccagggtttctgccattcattgagtttgccatctggaattttagttctttcggcgccgtagctgtccagagacacgcgtgtgcgcgggtcccactccacacgcacgcagcccagtgtgtgtggggagccccggctgggagtgggatcgctgagaacagctcgctcccgaagaaggagcaacccagcgcgcaggcctccgagacgtggaaacgcaacaattaccgtcaagacaaatccacacccgctctcccctcccgcccgactcggggaggccgcgggacgccgcagcagcactagcaggaggaggagaccgctcgctggac

SEQ ID NO: 9428 - RNA, 5639 nt, Homo sapiens
  source 1..5639: mol_type = other RNA
aggaggcatcttgagaaatggaaggaatgtctaactttttggatcacagtgaaacaaagtctggatcacttccagacatcaacgagcagtcgcttttacaataaaaaaaaatttttttaggtttaatttcataggtgatagatagcaatgggtctttcttgacagtgtttaatagaaagttttcctcttttcattccattacgtatgaatttttgattcattctttttaaatgacaatactaatggttgctattgagtacaagatgcagagattttgctggaggctggtaaattttctctgcaaaacagatatccccccaccccccacccccaaatttcaggtccaggtttgctatatcatcactagtccttttttaattctcactggaaattttcaaatattgtttataaactgaatgagaatgtgctatgttctctaacattcttattttacatcattctctaatatattaggaatgttgcaacaatgttatcacaatgaagtggcaacttttggcctttagactgtacctatcatcagcaatcataaaaaggccaaaataaacagtgctattccaaggtgacatctgaaactgttaaaacaagtgaaaaatcataatgacaaaacaggggttcataaagcaaaagaaaatttgccaatgcaattttaaaagtgtaagaaacttcactcatgtacctactcatgggaagaacatctaaggcaaatgaaaaattcccctccagggacataaccagctcagaaccatctgaaaaaattcatacaaaagcagaaattacccaaggcctgtgagtcctcatctcataccatgaaagccagactgtcaaaaaaagggcacatgtcactttgcaaaggaatgtattaactcctctcccagggtcaacttagtctacgtgtcttttgtataacattaatttccaccagatctactagatgttcagtcatgtcctttcaggtcctgaaggcaggctcactctctgatgcatctttttatatcatggtgggtgtgaagtgaaaagaggagacacagaaatatgcacaaacccacaattagtccatatttagaaaactttctgtgggttcaagcatttacacagagatgattttatctcatttctccattaatttcccatttgaaatgaaaaccagctaattctaaattctaaagccctgggggaaaccttccaggctttgtctatcagacagactttgtcataaaaaacacagaaaaacaaaaataaaacattacgctggaatcagcttttgagagtttgtgctttaaaaacacagtgcctaacagcaccaagcatatcatagatgctcaataaatatttgtagatttattaagagtaataacatggtgtttaaagaaccaaccaccattttgtaaaataggcaaaactacattaatttctttcacctgatttgataaagcagtgtggagcaatgaatgagagaatctgcaaattaaatatgaactctaatttgattgcagagagaaaattactgagaactttgcaaaaaacattgccacagtagccttgacactcaacagtgcaacgaagagttaatgtttccactgcaatatgaactggttcccacagctcttaggagatagagtgtaatcacttaaatgggaaatgaactctaattccacttgagaaaaggtatgttatgttcataattttatctgaaaattattaatatatttcagggagatggtcctctcattcagcatccctcaaagtaatgcaggcataagtatcaggggaccttgttatataacttcagtacagcattgtcttatacaagtgttctctcttccacatctgtagtagctgctttctaatattgtagatttttacagttgtgacacccctgggatgacagacatgagaatatggaggattaaaggttacaaaacttaaacaaaaaagggaagctcctctatgttatgtgaaaaccccttacaaaaggcagtttattgacaaataaatgctttatacattcaggtttttcccatctctcaatagtgatggtttccaaagaagaaactcagtagtgaagaatacatacttttttttttttgcattagtttgatcagttgaaaatcagaaccttcaaagcatcttgtgaatgagagaaatggaactggacctgggcaaggcatggggatggtagagatccatatgaataaatgatttagctgttgatgtggacagcaagagagttggtgggaaatgttacagcagacctgaccacgctacaaagggtctgtgaagaacacagtacaggtatcaaaacaccaaaacaaaactaaactaaaaacaagaacaaactgcaactttgccaaactgtaaacaaggtaaagcatttcacaggttcaaagttcaagggaagtaaacgtctttaaattatttttgtcagttcaaccctgatttaaaaatatggctagcaaaaacaaggaagccacagctgtcgacatcctgagcaagcatcggtctcctttgagaagctgcactcccaagcctcttctcaagctgctacacgaggaggagacacttctctcttgaattccatctcagttctctttatttccacactcttggaatacatcgattgctttccattttggtgtctacagttctggctgctatagatttagacgtggggatactggaggagggaaggcaaattctcggaggatgctccgggcaacttcgacattattctgggctatctctaaggctctcttcacctcttcaaaggcataaccctctcccatgagttttgcaatttttgcatcgacattttccaatgccgcctcaggcccatggggttttctgtggtgaatttctggtgcagtcctgcgcggtcgtggtttagggggtctggctggtgcctgtgaaccatctgaacatgaaggaagctgatcatagtcctgtgatgttctgttagttttgacattttcacctggtaaccttctagcaggaggcaaaggaacttggccacttgctagatcaacaaagggatctgaaggaagaagaaaaagatcctgtcctgaggatggccggctactggagccaggaggttttgaatgttcaatgagactatgccttgcaggaggtgggggaggtgggagagatggagggagggcatcaaaagcatcttcacctaatggagggatgagaagatcataatcagagggcgtcctgttgagtgaagaaccatgctttggattgtcccgagttggaggcctggcaggtggtaatggcacgggatcagaggctgaatcaaaaacatctccctttaaatatatgcttaagtcagggatgtttgatttcttctctgaagatggaccatgtgttccattcagcatacagtgaccattatcacaagactttatgctagggaggagggtggtaactggaggaggaggagaaagccggggaggaacatcatattcttcacttccaaggtgaccattggaaaagaccttagctccttctaaaggcaaatcatggcgtctgtgtttccgcataagcactgggtcagagcccactctactgtgccttccattgacatttgaactcgctgtgattccaggttttggagagccctcccctaggagtcgacatcccacaagctgattagtcccaaacacatcccgagggcaccatgcttcaagaggcattggcgggtctctggaaggcacgctttccacatgatggatgtgtctactcagtctattgtctggtgggattggtggaggtctttcaggtggcggtggaggaggatctcttaagggaggaggtggtgctgggagtggtttatcttgttttctcaccatgcaaggagaagactttggtgaacccgttgggctgccacagggagatctaactatgcctttctgaattagatccaggcgaggaggcacgggtggcaggcttagatgtgggatctggagtgggtcaggctgtggctttcttctctgggcaaggggagaggatcctggtgatgtgactggtgagttctgcctgtcagtgcactttcggacgtttgccaaccgattcatcatcaaggactcctcacgatcatcatcgtcgtccaagtctagcatcggcatgccaaaggggtcaatgatgctgcaacacctggagccttcatctcttggatcaaaggggtccacgattatgggctcagttccttttatttcacaacgacagaaagggcagccctgaccatccgactcctgccatgccgtaaggcaagaggtgcacatcaaatgcccacaaggctcaatcttgacatctttgtcattctctgcacaaatcttacagagctgaaaagtggagcccatttcacaatataattcatattgttcctgtgtaacttttatatggtcatgaggtgtaggttcacataatccagttaaatcaggattataactcctcccatcaggataaagataaaatccttccctgctgccatcaatcagggcttgaaataagggcttgttatgaggtatggtctgtaagatattcccatccccagtcacatagccaatggcccactgtcccaatcgagtgcaacttaaccggaaaatatagcttccgggtttggtgctatatttctgtagtcgtgctttaacttcatcatatgtgagaaatgccatgtaacctggatgtgtcacagctaagaaattccaattccgcaaaatagagccccaaggctgaaacagcctggtaaaaatatcaaattcaaaaactgaaatgtaatcattgcaagttaaatcaattgttgattttagagccattgcttccaggccagagctaatctggtggacctcatgaaggcactgtctgaatactttccatggtacgatagttttgtctccaaaaaactttctccagaattcagcagcatctgcttttgtgatacgaaagttatctccctggaattgaccattgggaaagattgctttgatttctgccagcatgtgactgaagataagggacagttttgtgagatttcgtctgtcctgtgactgttcttcatacattctctccttgccttctttaaagagtcttattgcccgttttgactttttcataaggctatcaatgtagattttaaagtactcattctcactgagttgggcaagtttctggttgtcatcatatttactcaatataagtcgtaaatgctgatatgtatcaggcaaaatatcaagtatatatggtgggctatttttcaactgaagtttgggattttggcacagtcttaccactttgtccatgagcttccaagtcttctccacggtcctgcgatctgcggcagcttgcttagggggtccaactgcatcctgaatagcatcaataatacccaaaattcgaccttttcggggatttcctcctcgaccaccagggtttctgccattcattgagtttgccatctggaattttagttctttctttaaatcaacgcggtgagtcgttattcccaagaaccaaatgaaattaacacacaaatagcccatttgaaaagagaaaagagaaaaatgacaagagcggccacggaaaggaggagttcacttctctggctcctcgcctctgccctc

SEQ ID NO: 9429 - RNA, 5677 nt, Homo sapiens
  source 1..5677: mol_type = other RNA
aggaggcatcttgagaaatggaaggaatgtctaactttttggatcacagtgaaacaaagtctggatcacttccagacatcaacgagcagtcgcttttacaataaaaaaaaatttttttaggtttaatttcataggtgatagatagcaatgggtctttcttgacagtgtttaatagaaagttttcctcttttcattccattacgtatgaatttttgattcattctttttaaatgacaatactaatggttgctattgagtacaagatgcagagattttgctggaggctggtaaattttctctgcaaaacagatatccccccaccccccacccccaaatttcaggtccaggtttgctatatcatcactagtccttttttaattctcactggaaattttcaaatattgtttataaactgaatgagaatgtgctatgttctctaacattcttattttacatcattctctaatatattaggaatgttgcaacaatgttatcacaatgaagtggcaacttttggcctttagactgtacctatcatcagcaatcataaaaaggccaaaataaacagtgctattccaaggtgacatctgaaactgttaaaacaagtgaaaaatcataatgacaaaacaggggttcataaagcaaaagaaaatttgccaatgcaattttaaaagtgtaagaaacttcactcatgtacctactcatgggaagaacatctaaggcaaatgaaaaattcccctccagggacataaccagctcagaaccatctgaaaaaattcatacaaaagcagaaattacccaaggcctgtgagtcctcatctcataccatgaaagccagactgtcaaaaaaagggcacatgtcactttgcaaaggaatgtattaactcctctcccagggtcaacttagtctacgtgtcttttgtataacattaatttccaccagatctactagatgttcagtcatgtcctttcaggtcctgaaggcaggctcactctctgatgcatctttttatatcatggtgggtgtgaagtgaaaagaggagacacagaaatatgcacaaacccacaattagtccatatttagaaaactttctgtgggttcaagcatttacacagagatgattttatctcatttctccattaatttcccatttgaaatgaaaaccagctaattctaaattctaaagccctgggggaaaccttccaggctttgtctatcagacagactttgtcataaaaaacacagaaaaacaaaaataaaacattacgctggaatcagcttttgagagtttgtgctttaaaaacacagtgcctaacagcaccaagcatatcatagatgctcaataaatatttgtagatttattaagagtaataacatggtgtttaaagaaccaaccaccattttgtaaaataggcaaaactacattaatttctttcacctgatttgataaagcagtgtggagcaatgaatgagagaatctgcaaattaaatatgaactctaatttgattgcagagagaaaattactgagaactttgcaaaaaacattgccacagtagccttgacactcaacagtgcaacgaagagttaatgtttccactgcaatatgaactggttcccacagctcttaggagatagagtgtaatcacttaaatgggaaatgaactctaattccacttgagaaaaggtatgttatgttcataattttatctgaaaattattaatatatttcagggagatggtcctctcattcagcatccctcaaagtaatgcaggcataagtatcaggggaccttgttatataacttcagtacagcattgtcttatacaagtgttctctcttccacatctgtagtagctgctttctaatattgtagatttttacagttgtgacacccctgggatgacagacatgagaatatggaggattaaaggttacaaaacttaaacaaaaaagggaagctcctctatgttatgtgaaaaccccttacaaaaggcagtttattgacaaataaatgctttatacattcaggtttttcccatctctcaatagtgatggtttccaaagaagaaactcagtagtgaagaatacatacttttttttttttgcattagtttgatcagttgaaaatcagaaccttcaaagcatcttgtgaatgagagaaatggaactggacctgggcaaggcatggggatggtagagatccatatgaataaatgatttagctgttgatgtggacagcaagagagttggtgggaaatgttacagcagacctgaccacgctacaaagggtctgtgaagaacacagtacaggtatcaaaacaccaaaacaaaactaaactaaaaacaagaacaaactgcaactttgccaaactgtaaacaaggtaaagcatttcacaggttcaaagttcaagggaagtaaacgtctttaaattatttttgtcagttcaaccctgatttaaaaatatggctagcaaaaacaaggaagccacagctgtcgacatcctgagcaagcatcggtctcctttgagaagctgcactcccaagcctcttctcaagctgctacacgaggaggagacacttctctcttgaattccatctcagttctctttatttccacactcttggaatacatcgattgctttccattttggtgtctacagttctggctgctatagatttagacgtggggatactggaggagggaaggcaaattctcggaggatgctccgggcaacttcgacattattctgggctatctctaaggctctcttcacctcttcaaaggcataaccctctcccatgagttttgcaatttttgcatcgacattttccaatgccgcctcaggcccatggggttttctgtggtgaatttctggtgcagtcctgcgcggtcgtggtttagggggtctggctggtgcctgtgaaccatctgaacatgaaggaagctgatcatagtcctgtgatgttctgttagttttgacattttcacctggtaaccttctagcaggaggcaaaggaacttggccacttgctagatcaacaaagggatctgaaggaagaagaaaaagatcctgtcctgaggatggccggctactggagccaggaggttttgaatgttcaatgagactatgccttgcaggaggtgggggaggtgggagagatggagggagggcatcaaaagcatcttcacctaatggagggatgagaagatcataatcagagggcgtcctgttgagtgaagaaccatgctttggattgtcccgagttggaggcctggcaggtggtaatggcacgggatcagaggctgaatcaaaaacatctccctttaaatatatgcttaagtcagggatgtttgatttcttctctgaagatggaccatgtgttccattcagcatacagtgaccattatcacaagactttatgctagggaggagggtggtaactggaggaggaggagaaagccggggaggaacatcatattcttcacttccaaggtgaccattggaaaagaccttagctccttctaaaggcaaatcatggcgtctgtgtttccgcataagcactgggtcagagcccactctactgtgccttccattgacatttgaactcgctgtgattccaggttttggagagccctcccctaggagtcgacatcccacaagctgattagtcccaaacacatcccgagggcaccatgcttcaagaggcattggcgggtctctggaaggcacgctttccacatgatggatgtgtctactcagtctattgtctggtgggattggtggaggtctttcaggtggcggtggaggaggatctcttaagggaggaggtggtgctgggagtggtttatcttgttttctcaccatgcaaggagaagactttggtgaacccgttgggctgccacagggagatctaactatgcctttctgaattagatccaggcgaggaggcacgggtggcaggcttagatgtgggatctggagtgggtcaggctgtggctttcttctctgggcaaggggagaggatcctggtgatgtgactggtgagttctgcctgtcagtgcactttcggacgtttgccaaccgattcatcatcaaggactcctcacgatcatcatcgtcgtccaagtctagcatcggcatgccaaaggggtcaatgatgctgcaacacctggagccttcatctcttggatcaaaggggtccacgattatgggctcagttccttttatttcacaacgacagaaagggcagccctgaccatccgactcctgccatgccgtaaggcaagaggtgcacatcaaatgcccacaaggctcaatcttgacatctttgtcattctctgcacaaatcttacagagctgaaaagtggagcccatttcacaatataattcatattgttcctgtgtaacttttatatggtcatgaggtgtaggttcacataatccagttaaatcaggattataactcctcccatcaggataaagataaaatccttccctgctgccatcaatcagggcttgaaataagggcttgttatgaggtatggtctgtaagatattcccatccccagtcacatagccaatggcccactgtcccaatcgagtgcaacttaaccggaaaatatagcttccgggtttggtgctatatttctgtagtcgtgctttaacttcatcatatgtgagaaatgccatgtaacctggatgtgtcacagctaagaaattccaattccgcaaaatagagccccaaggttcctagaatgagcagttaggtttaatgtaggaagattacttttactctcttccttgacaaggtgaagaagcaaagctcttactatttagaatgtctttgtatcatgttaaataaataagatattctgtaaaattatcagaaacctgaaacagcctggtaaaaatatcaaattcaaaaactgaaatgtaatcattgcaagttaaatcaattgttgattttagagccattgcttccaggccagagctaatctggtggacctcatgaaggcactgtctgaatactttccatggtacgatagttttgtctccaaaaaactttctccagaattcagcagcatctgcttttgtgatacgaaagttatctccctggaattgaccattgggaaagattgctttgatttctgccagcatgtgactgaagataagggacagttttgtgagatttcgtcattttttttgcctttagaagatcacaatggtaattcacaaagaactgtcctgtgactgttcttcatacattctctccttgccttctttaaagagtcttattgcccgttttgactttttcataaggctatcaatgtagattttaaagtactcattctcactgagttgggcaagtttctggttgtcatcatatttactcaatataagtcgtaaatgctgatatgtatcaggcaaaatatcaagtatatatggtgggctatttttcaactgaagtttgggattttggcacagtcttaccactttgtccatgagcttccaagtcttctccacggtcctgcgatctgcggcagcttgcttagggggtccaactgcatcctgaatagcatcaataatacccaaaattcgaccttttcggggatttcctcctcgaccaccagggtttctgccattcattgagtttgccatctggaattttagtt

SEQ ID NO: 9430 - RNA, 5608 nt, Homo sapiens
  source 1..5608: mol_type = other RNA
aggaggcatcttgagaaatggaaggaatgtctaactttttggatcacagtgaaacaaagtctggatcacttccagacatcaacgagcagtcgcttttacaataaaaaaaaatttttttaggtttaatttcataggtgatagatagcaatgggtctttcttgacagtgtttaatagaaagttttcctcttttcattccattacgtatgaatttttgattcattctttttaaatgacaatactaatggttgctattgagtacaagatgcagagattttgctggaggctggtaaattttctctgcaaaacagatatccccccaccccccacccccaaatttcaggtccaggtttgctatatcatcactagtccttttttaattctcactggaaattttcaaatattgtttataaactgaatgagaatgtgctatgttctctaacattcttattttacatcattctctaatatattaggaatgttgcaacaatgttatcacaatgaagtggcaacttttggcctttagactgtacctatcatcagcaatcataaaaaggccaaaataaacagtgctattccaaggtgacatctgaaactgttaaaacaagtgaaaaatcataatgacaaaacaggggttcataaagcaaaagaaaatttgccaatgcaattttaaaagtgtaagaaacttcactcatgtacctactcatgggaagaacatctaaggcaaatgaaaaattcccctccagggacataaccagctcagaaccatctgaaaaaattcatacaaaagcagaaattacccaaggcctgtgagtcctcatctcataccatgaaagccagactgtcaaaaaaagggcacatgtcactttgcaaaggaatgtattaactcctctcccagggtcaacttagtctacgtgtcttttgtataacattaatttccaccagatctactagatgttcagtcatgtcctttcaggtcctgaaggcaggctcactctctgatgcatctttttatatcatggtgggtgtgaagtgaaaagaggagacacagaaatatgcacaaacccacaattagtccatatttagaaaactttctgtgggttcaagcatttacacagagatgattttatctcatttctccattaatttcccatttgaaatgaaaaccagctaattctaaattctaaagccctgggggaaaccttccaggctttgtctatcagacagactttgtcataaaaaacacagaaaaacaaaaataaaacattacgctggaatcagcttttgagagtttgtgctttaaaaacacagtgcctaacagcaccaagcatatcatagatgctcaataaatatttgtagatttattaagagtaataacatggtgtttaaagaaccaaccaccattttgtaaaataggcaaaactacattaatttctttcacctgatttgataaagcagtgtggagcaatgaatgagagaatctgcaaattaaatatgaactctaatttgattgcagagagaaaattactgagaactttgcaaaaaacattgccacagtagccttgacactcaacagtgcaacgaagagttaatgtttccactgcaatatgaactggttcccacagctcttaggagatagagtgtaatcacttaaatgggaaatgaactctaattccacttgagaaaaggtatgttatgttcataattttatctgaaaattattaatatatttcagggagatggtcctctcattcagcatccctcaaagtaatgcaggcataagtatcaggggaccttgttatataacttcagtacagcattgtcttatacaagtgttctctcttccacatctgtagtagctgctttctaatattgtagatttttacagttgtgacacccctgggatgacagacatgagaatatggaggattaaaggttacaaaacttaaacaaaaaagggaagctcctctatgttatgtgaaaaccccttacaaaaggcagtttattgacaaataaatgctttatacattcaggtttttcccatctctcaatagtgatggtttccaaagaagaaactcagtagtgaagaatacatacttttttttttttgcattagtttgatcagttgaaaatcagaaccttcaaagcatcttgtgaatgagagaaatggaactggacctgggcaaggcatggggatggtagagatccatatgaataaatgatttagctgttgatgtggacagcaagagagttggtgggaaatgttacagcagacctgaccacgctacaaagggtctgtgaagaacacagtacaggtatcaaaacaccaaaacaaaactaaactaaaaacaagaacaaactgcaactttgccaaactgtaaacaaggtaaagcatttcacaggttcaaagttcaagggaagtaaacgtctttaaattatttttgtcagttcaaccctgatttaaaaatatggctagcaaaaacaaggaagccacagctgtcgacatcctgagcaagcatcggtctcctttgagaagctgcactcccaagcctcttctcaagctgctacacgaggaggagacacttctctcttgaattccatctcagttctctttatttccacactcttggaatacatcgattgctttccattttggtgtctacagttctggctgctatagatttagacgtggggatactggaggagggaaggcaaattctcggaggatgctccgggcaacttcgacattattctgggctatctctaaggctctcttcacctcttcaaaggcataaccctctcccatgagttttgcaatttttgcatcgacattttccaatgccgcctcaggcccatggggttttctgtggtgaatttctggtgcagtcctgcgcggtcgtggtttagggggtctggctggtgcctgtgaaccatctgaacatgaaggaagctgatcatagtcctgtgatgttctgttagttttgacattttcacctggtaaccttctagcaggaggcaaaggaacttggccacttgctagatcaacaaagggatctgaaggaagaagaaaaagatcctgtcctgaggatggccggctactggagccaggaggttttgaatgttcaatgagactatgccttgcaggaggtgggggaggtgggagagatggagggagggcatcaaaagcatcttcacctaatggagggatgagaagatcataatcagagggcgtcctgttgagtgaagaaccatgctttggattgtcccgagttggaggcctggcaggtggtaatggcacgggatcagaggctgaatcaaaaacatctccctttaaatatatgcttaagtcagggatgtttgatttcttctctgaagatggaccatgtgttccattcagcatacagtgaccattatcacaagactttatgctagggaggagggtggtaactggaggaggaggagaaagccggggaggaacatcatattcttcacttccaaggtgaccattggaaaagaccttagctccttctaaaggcaaatcatggcgtctgtgtttccgcataagcactgggtcagagcccactctactgtgccttccattgacatttgaactcgctgtgattccaggttttggagagccctcccctaggagtcgacatcccacaagctgattagtcccaaacacatcccgagggcaccatgcttcaagaggcattggcgggtctctggaaggcacgctttccacatgatggatgtgtctactcagtctattgtctggtgggattggtggaggtctttcaggtggcggtggaggaggatctcttaagggaggaggtggtgctgggagtggtttatcttgttttctcaccatgcaaggagaagactttggtgaacccgttgggctgccacagggagatctaactatgcctttctgaattagatccaggcgaggaggcacgggtggcaggcttagatgtgggatctggagtgggtcaggctgtggctttcttctctgggcaaggggagaggatcctggtgatgtgactggtgagttctgcctgtcagtgcactttcggacgtttgccaaccgattcatcatcaaggactcctcacgatcatcatcgtcgtccaagtctagcatcggcatgccaaaggggtcaatgatgctgcaacacctggagccttcatctcttggatcaaaggggtccacgattatgggctcagttccttttatttcacaacgacagaaagggcagccctgaccatccgactcctgccatgccgtaaggcaagaggtgcacatcaaatgcccacaaggctcaatcttgacatctttgtcattctctgcacaaatcttacagagctgaaaagtggagcccatttcacaatataattcatattgttcctgtgtaacttttatatggtcatgaggtgtaggttcacataatccagttaaatcaggattataactcctcccatcaggataaagataaaatccttccctgctgccatcaatcagggcttgaaataagggcttgttatgaggtatggtctgtaagatattcccatccccagtcacatagccaatggcccactgtcccaatcgagtgcaacttaaccggaaaatatagcttccgggtttggtgctatatttctgtagtcgtgctttaacttcatcatatgtgagaaatgccatgtaacctggatgtgtcacagctaagaaattccaattccgcaaaatagagccccaaggttgtctccaaaaaactttctccagaattcagcagcatctgcttttgtgatacgaaagttatctccctggaattgaccattgggaaagattgctttgatttctgccagcatgtgactgaagataagggacagttttgtgagatttcgtctgtcctgtgactgttcttcatacattctctccttgccttctttaaagagtcttattgcccgttttgactttttcataaggctatcaatgtagattttaaagtactcattctcactgagttgggcaagtttctggttgtcatcatatttactcaatataagtcgtaaatgctgatatgtatcaggcaaaatatcaagtatatatggtgggctatttttcaactgaagtttgggattttggcacagtcttaccactttgtccatgagcttccaagtcttctccacggtcctgcgatctgcggcagcttgcttagggggtccaactgcatcctgaatagcatcaataatacccaaaattcgaccttttcggggatttcctcctcgaccaccagggtttctgccattcattgagtttgccatctggaattttagttctttcggcgccgtagctgtccagagacacgcgtgtgcgcgggtcccactccacacgcacgcagcccagtgtgtgtggggagccccggctgggagtgggatcgctgagaacagctcgctcccgaagaaggagcaacccagcgcgcaggcctccgagacgtggaaacgcaacaattaccgtcaagacaaatccacacccgctctcccctcccgcccgactcggggaggccgcgggacgccgcagcagcactagcaggaggaggagaccgctcgctggac

SEQ ID NO: 9431 - RNA, 6137 nt, Homo sapiens
  source 1..6137: mol_type = other RNA
aggaggcatcttgagaaatggaaggaatgtctaactttttggatcacagtgaaacaaagtctggatcacttccagacatcaacgagcagtcgcttttacaataaaaaaaaatttttttaggtttaatttcataggtgatagatagcaatgggtctttcttgacagtgtttaatagaaagttttcctcttttcattccattacgtatgaatttttgattcattctttttaaatgacaatactaatggttgctattgagtacaagatgcagagattttgctggaggctggtaaattttctctgcaaaacagatatccccccaccccccacccccaaatttcaggtccaggtttgctatatcatcactagtccttttttaattctcactggaaattttcaaatattgtttataaactgaatgagaatgtgctatgttctctaacattcttattttacatcattctctaatatattaggaatgttgcaacaatgttatcacaatgaagtggcaacttttggcctttagactgtacctatcatcagcaatcataaaaaggccaaaataaacagtgctattccaaggtgacatctgaaactgttaaaacaagtgaaaaatcataatgacaaaacaggggttcataaagcaaaagaaaatttgccaatgcaattttaaaagtgtaagaaacttcactcatgtacctactcatgggaagaacatctaaggcaaatgaaaaattcccctccagggacataaccagctcagaaccatctgaaaaaattcatacaaaagcagaaattacccaaggcctgtgagtcctcatctcataccatgaaagccagactgtcaaaaaaagggcacatgtcactttgcaaaggaatgtattaactcctctcccagggtcaacttagtctacgtgtcttttgtataacattaatttccaccagatctactagatgttcagtcatgtcctttcaggtcctgaaggcaggctcactctctgatgcatctttttatatcatggtgggtgtgaagtgaaaagaggagacacagaaatatgcacaaacccacaattagtccatatttagaaaactttctgtgggttcaagcatttacacagagatgattttatctcatttctccattaatttcccatttgaaatgaaaaccagctaattctaaattctaaagccctgggggaaaccttccaggctttgtctatcagacagactttgtcataaaaaacacagaaaaacaaaaataaaacattacgctggaatcagcttttgagagtttgtgctttaaaaacacagtgcctaacagcaccaagcatatcatagatgctcaataaatatttgtagatttattaagagtaataacatggtgtttaaagaaccaaccaccattttgtaaaataggcaaaactacattaatttctttcacctgatttgataaagcagtgtggagcaatgaatgagagaatctgcaaattaaatatgaactctaatttgattgcagagagaaaattactgagaactttgcaaaaaacattgccacagtagccttgacactcaacagtgcaacgaagagttaatgtttccactgcaatatgaactggttcccacagctcttaggagatagagtgtaatcacttaaatgggaaatgaactctaattccacttgagaaaaggtatgttatgttcataattttatctgaaaattattaatatatttcagggagatggtcctctcattcagcatccctcaaagtaatgcaggcataagtatcaggggaccttgttatataacttcagtacagcattgtcttatacaagtgttctctcttccacatctgtagtagctgctttctaatattgtagatttttacagttgtgacacccctgggatgacagacatgagaatatggaggattaaaggttacaaaacttaaacaaaaaagggaagctcctctatgttatgtgaaaaccccttacaaaaggcagtttattgacaaataaatgctttatacattcaggtttttcccatctctcaatagtgatggtttccaaagaagaaactcagtagtgaagaatacatacttttttttttttgcattagtttgatcagttgaaaatcagaaccttcaaagcatcttgtgaatgagagaaatggaactggacctgggcaaggcatggggatggtagagatccatatgaataaatgatttagctgttgatgtggacagcaagagagttggtgggaaatgttacagcagacctgaccacgctacaaagggtctgtgaagaacacagtacaggtatcaaaacaccaaaacaaaactaaactaaaaacaagaacaaactgcaactttgccaaactgtaaacaaggtaaagcatttcacaggttcaaagttcaagggaagtaaacgtctttaaattatttttgtcagttcaaccctgatttaaaaatatggctagcaaaaacaaggaagccacagctgtcgacatcctgagcaagcatcggtctcctttgagaagctgcactcccaagcctcttctcaagctgctacacgaggaggagacacttctctcttgaattccatctcagttctctttatttccacactcttggaatacatcgattgctttccattttggtgtctacagttctggctgctatagatttagacgtggggatactggaggagggaaggcaaattctcggaggatgctccgggcaacttcgacattattctgggctatctctaaggctctcttcacctcttcaaaggcataaccctctcccatgagttttgcaatttttgcatcgacattttccaatgccgcctcaggcccatggggttttctgtggtgaatttctggtgcagtcctgcgcggtcgtggtttagggggtctggctggtgcctgtgaaccatctgaacatgaaggaagctgatcatagtcctgtgatgttctgttagttttgacattttcacctggtaaccttctagcaggaggcaaaggaacttggccacttgctagatcaacaaagggatctgcttatggttctgttttgaatcattatcatgttctatcttgcatcatatcctaagtttgctatttgtcagccatagggtaaactgggctctctgaaggaagaagaaaaagatcctgtcctgaggatggccggctactggagccaggaggttttgaatgttcaatgagactatgccttgcaggaggtgggggaggtgggagagatggagggagggcatcaaaagcatcttcacctaatggagggatgagaagatcataatcagagggcgtcctgttgagtgaagaaccatgctttggattgtcccgagttggaggcctggcaggtggtaatggcacgggatcagaggctgaatcaaaaacatctccctttaaatatatgcttaagtcagggatgtttgatttcttctctgaagatggaccatgtgttccattcagcatacagtgaccattatcacaagaccgaacaggaggttttacattatgacaatgagatggttgtgaattcagggaaacagggtgggatgaaggaatcttgtattcatcatcatcttcctctactgggtctcttgttttctctgaaagagaatttgctaacggaccagtacactttatgctagggaggagggtggtaactggaggaggaggagaaagccggggaggaacatcatattcttcacttccaaggtgaccattggaaaagaccttagctccttctaaaggcaaatcatggcgtctgtgtttccgcataagcactgggtcagagcccactctactgtgccttccattgacatttgaactcgctgtgattccaggttttggagagccctcccctaggagtcgacatcccacaagctgattagtcccaaacacatcccgagggcaccatgcttcaagaggcattggcgggtctctggaaggcacgctttccacatgatggatgtgtctactcagtctattgtctggtgggattggtggaggtctttcaggtggcggtggaggaggatctcttaagggaggaggtggtgctgggagtggtttatcttgttttctcaccatgcaaggagaagactttggtgaacccgttgggctgccacagggagatctaactatgcctttctgaattagatccaggcgaggaggcacgggtggcaggcttagatgtgggatctggagtgggtcaggctgtggctttcttctctgggcaaggggagaggatcctggtgatgtgactggtgagttctgcctgtcagtgcactttcggacgtttgccaaccgattcatcatcaaggactcctcacgatcatcatcgtcgtccaagtctagcatcggcatgccaaaggggtcaatgatgctgcaacacctggagccttcatctcttggatcaaaggggtccacgattatgggctcagttccttttatttcacaacgacagaaagggcagccctgaccatccgactcctgccatgccgtaaggcaagaggtgcacatcaaatgcccacaaggctcaatcttgacatctttgtcattctctgcacaaatcttacagagctgaaaagtggagcccatttcacaatataattcatattgttcctgtgtaacttttatatggtcatgaggtgtaggttcacataatccagttaaatcaggattataactcctcccatcaggataaagataaaatccttccctgctgccatcaatcagggcttgaaataagggcttgttatgaggtatggtctgtaagatattcccatccccagtcacatagccaatggcccactgtcccaatcgagtgcaacttaaccggaaaatatagcttccgggtttggtgctatatttctgtagtcgtgctttaacttcatcatatgtgagaaatgccatgtaacctggatgtgtcacagctaagaaattccaattccgcaaaatagagccccaaggctgaaacagcctggtaaaaatatcaaattcaaaaactgaaatgtaatcattgcaagttaaatcaattgttgattttagagccattgcttccaggccagagctaatctggtggacctcatgaaggcactgtctgaatactttccatggtacgatagttctccatttaaacttctgcaaaaagacagtggtggtttctactacctcttcctttagagatgaagcaaatgagagaaaatatcaatagcaaattgttttacaaatgtagaaatttcagggtgctggcagagacttgtctccaaaaaactttctccagaattcagcagcatctgcttttgtgatacgaaagttatctccctggaattgaccattgggaaagattgctttgatttctgccagcatgtgactgaagataagggacagttttgtgagatttcgtctgtcctgtgactgttcttcatacattctctccttgccttctttaaagagtcttattgcccgttttgactttttcataaggctatcaatgtagattttaaagtactcattctcactgagttgggcaagtttctggttgtcatcatatttactcaatataagtcgtaaatgctgatatgtatcaggcaaaatatcaagtatatatggtgggctatttttcaactgaagtttgggattttggcacagtcttaccactttgtccatgagcttccaagtcttctccacggtcctgcgatctgcggcagcttgcttagggggtccaactgcatcctgaatagcatcaataatacccaaaattcgaccttttcggggatttcctcctcgaccaccagggtttctgccattcattgagtttgccatctggaattttagttctttcggcgccgtagctgtccagagacacgcgtgtgcgcgggtcccactccacacgcacgcagcccagtgtgtgtggggagccccggctgggagtgggatcgctgagaacagctcgctcccgaagaaggagcaacccagcgcgcaggcctccgagacgtggaaacgcaacaattaccgtcaagacaaatccacacccgctctcccctcccgcccgactcggggaggccgcgggacgccgcagcagcactagcaggaggaggagaccgctcgctggac

SEQ ID NO: 9432 - RNA, 5649 nt, Homo sapiens
  source 1..5649: mol_type = other RNA
aggaggcatcttgagaaatggaaggaatgtctaactttttggatcacagtgaaacaaagtctggatcacttccagacatcaacgagcagtcgcttttacaataaaaaaaaatttttttaggtttaatttcataggtgatagatagcaatgggtctttcttgacagtgtttaatagaaagttttcctcttttcattccattacgtatgaatttttgattcattctttttaaatgacaatactaatggttgctattgagtacaagatgcagagattttgctggaggctggtaaattttctctgcaaaacagatatccccccaccccccacccccaaatttcaggtccaggtttgctatatcatcactagtccttttttaattctcactggaaattttcaaatattgtttataaactgaatgagaatgtgctatgttctctaacattcttattttacatcattctctaatatattaggaatgttgcaacaatgttatcacaatgaagtggcaacttttggcctttagactgtacctatcatcagcaatcataaaaaggccaaaataaacagtgctattccaaggtgacatctgaaactgttaaaacaagtgaaaaatcataatgacaaaacaggggttcataaagcaaaagaaaatttgccaatgcaattttaaaagtgtaagaaacttcactcatgtacctactcatgggaagaacatctaaggcaaatgaaaaattcccctccagggacataaccagctcagaaccatctgaaaaaattcatacaaaagcagaaattacccaaggcctgtgagtcctcatctcataccatgaaagccagactgtcaaaaaaagggcacatgtcactttgcaaaggaatgtattaactcctctcccagggtcaacttagtctacgtgtcttttgtataacattaatttccaccagatctactagatgttcagtcatgtcctttcaggtcctgaaggcaggctcactctctgatgcatctttttatatcatggtgggtgtgaagtgaaaagaggagacacagaaatatgcacaaacccacaattagtccatatttagaaaactttctgtgggttcaagcatttacacagagatgattttatctcatttctccattaatttcccatttgaaatgaaaaccagctaattctaaattctaaagccctgggggaaaccttccaggctttgtctatcagacagactttgtcataaaaaacacagaaaaacaaaaataaaacattacgctggaatcagcttttgagagtttgtgctttaaaaacacagtgcctaacagcaccaagcatatcatagatgctcaataaatatttgtagatttattaagagtaataacatggtgtttaaagaaccaaccaccattttgtaaaataggcaaaactacattaatttctttcacctgatttgataaagcagtgtggagcaatgaatgagagaatctgcaaattaaatatgaactctaatttgattgcagagagaaaattactgagaactttgcaaaaaacattgccacagtagccttgacactcaacagtgcaacgaagagttaatgtttccactgcaatatgaactggttcccacagctcttaggagatagagtgtaatcacttaaatgggaaatgaactctaattccacttgagaaaaggtatgttatgttcataattttatctgaaaattattaatatatttcagggagatggtcctctcattcagcatccctcaaagtaatgcaggcataagtatcaggggaccttgttatataacttcagtacagcattgtcttatacaagtgttctctcttccacatctgtagtagctgctttctaatattgtagatttttacagttgtgacacccctgggatgacagacatgagaatatggaggattaaaggttacaaaacttaaacaaaaaagggaagctcctctatgttatgtgaaaaccccttacaaaaggcagtttattgacaaataaatgctttatacattcaggtttttcccatctctcaatagtgatggtttccaaagaagaaactcagtagtgaagaatacatacttttttttttttgcattagtttgatcagttgaaaatcagaaccttcaaagcatcttgtgaatgagagaaatggaactggacctgggcaaggcatggggatggtagagatccatatgaataaatgatttagctgttgatgtggacagcaagagagttggtgggaaatgttacagcagacctgaccacgctacaaagggtctgtgaagaacacagtacaggtatcaaaacaccaaaacaaaactaaactaaaaacaagaacaaactgcaactttgccaaactgtaaacaaggtaaagcatttcacaggttcaaagttcaagggaagtaaacgtctttaaattatttttgtcagttcaaccctgatttaaaaatatggctagcaaaaacaaggaagccacagctgtcgacatcctgagcaagcatcggtctcctttgagaagctgcactcccaagcctcttctcaagctgctacacgaggaggagacacttctctcttgaattccatctcagttctctttatttccacactcttggaatacatcgattgctttccattttggtgtctacagttctggctgctatagatttagacgtggggatactggaggagggaaggcaaattctcggaggatgctccgggcaacttcgacattattctgggctatctctaaggctctcttcacctcttcaaaggcataaccctctcccatgagttttgcaatttttgcatcgacattttccaatgccgcctcaggcccatggggttttctgtggtgaatttctggtgcagtcctgcgcggtcgtggtttagggggtctggctggtgcctgtgaaccatctgaacatgaaggaagctgatcatagtcctgtgatgttctgttagttttgacattttcacctggtaaccttctagcaggaggcaaaggaacttggccacttgctagatcaacaaagggatctgtaatcccagctacttagggggtagaggcaggagaatcacttgaaccttggaggcagaggttgcagtgaactgagatcgcaccactgtactccagcctgggcaacagagtgagaccctgaaggaagaagaaaaagatcctgtcctgaggatggccggctactggagccaggaggttttgaatgttcaatgagactatgccttgcaggaggtgggggaggtgggagagatggagggagggcatcaaaagcatcttcaccctttaaatatatgcttaagtcagggatgtttgatttcttctctgaagatggaccatgtgttccattcagcatacagtgaccattatcacaagaccgaacaggaggttttacattatgacaatgagatggttgtgaattcagggaaacagggtgggatgaaggaatcttgtattcatcatcatcttcctctactgggtctcttgttttctctgaaagagaatttgctaacggaccagtacactttatgctagggaggagggtggtaactggaggaggaggagaaagccggggaggaacatcatattcttcacttccaaggtgaccattggaaaagaccttagctccttctaaaggcaaatcatggcgtctgtgtttccgcataagcactgggtcagagcccactctactgtgccttccattgacatttgaactcgctgtgattccaggttttggagagccctcccctaggagtcgacatcccacaagctgattagtcccaaacacatcccgagggcaccatgcttcaagaggcattggcgggtctctggaaggcacgctttccacatgatggatgtgtctactcagtctattgtctggtgggattggtggaggtctttcaggtggcggtggaggaggatctcttaagggaggaggtggtgctgggagtggtttatcttgttttctcaccatgcaaggagaagactttggtgaacccgttgggctgccacagggagatctaactatgcctttctgaattagatccaggcgaggaggcacgggtggcaggcttagatgtgggatctggagtgggtcaggctgtggctttcttctctgggcaaggggagaggatcctggtgatgtgactggtgagttctgcctgtcagtgcactttcggacgtttgccaaccgattcatcatcaaggactcctcacgatcatcatcgtcgtccaagtctagcatcggcatgccaaaggggtcaatgatgctgcaacacctggagccttcatctcttggatcaaaggggtccacgattatgggctcagttccttttatttcacaacgacagaaagggcagccctgaccatccgactcctgccatgccgtaaggcaagaggtgcacatcaaatgcccacaaggctcaatcttgacatctttgtcattctctgcacaaatcttacagagctgaaaagtggagcccatttcacaatataattcatattgttcctgtgtaacttttatatggtcatgaggtgtaggttcacataatccagttaaatcaggattataactcctcccatcaggataaagataaaatccttccctgctgccatcaatcagggcttgaaataagggcttgttatgaggtatggtctgtaagatattcccatccccagtcacatagccaatggcccactgtcccaatcgagtgcaacttaaccggaaaatatagcttccgggtttggtgctatatttctgtagtcgtgctttaacttcatcatatgtgagaaatgccatgtaacctggatgtgtcacagctaagaaattccaattccgcaaaatagagccccaaggctgaaacagcctggtaaaaatatcaaattcaaaaactgaaatgtaatcattgcaagttaaatcaattgttgattttagagccattgcttccaggccagagctaatctggtggacctcatgaaggcactgtctgaatactttccatggtacgatagttttgtctccaaaaaactttctccagaattcagcagcatctgcttttgtgatacgaaagttatctccctggaattgaccattgggaaagattgctttgatttctgccagcatgtgactgaagataagggacagttttgtgagatttcgtctgtcctgtgactgttcttcatacattctctccttgccttctttaaagagtcttattgcccgttttgactttttcataaggctatcaatgtagattttaaagtactcattctcactgagttgggcaagtttctggttgtcatcatatttactcaatataagtcgtaaatgctgatatgtatcaggcaaaatatcaagtatatatggtgggctatttttcaactgaagtttgggattttggcacagtcttaccactttgtccatgagcttccaagtcttctccacggtcctgcgatctgcggcagcttgcttagggggtccaactgcatcctgaatagcatcaataatacccaaaattcgaccttttcggggatttcctcctcgaccaccagggtttctgccattcattgagtttgccatctggaattttagttcgccgtctgcctggacgccctctccctc

SEQ ID NO: 9433 - RNA, 5983 nt, Homo sapiens
  source 1..5983: mol_type = other RNA
aggaggcatcttgagaaatggaaggaatgtctaactttttggatcacagtgaaacaaagtctggatcacttccagacatcaacgagcagtcgcttttacaataaaaaaaaatttttttaggtttaatttcataggtgatagatagcaatgggtctttcttgacagtgtttaatagaaagttttcctcttttcattccattacgtatgaatttttgattcattctttttaaatgacaatactaatggttgctattgagtacaagatgcagagattttgctggaggctggtaaattttctctgcaaaacagatatccccccaccccccacccccaaatttcaggtccaggtttgctatatcatcactagtccttttttaattctcactggaaattttcaaatattgtttataaactgaatgagaatgtgctatgttctctaacattcttattttacatcattctctaatatattaggaatgttgcaacaatgttatcacaatgaagtggcaacttttggcctttagactgtacctatcatcagcaatcataaaaaggccaaaataaacagtgctattccaaggtgacatctgaaactgttaaaacaagtgaaaaatcataatgacaaaacaggggttcataaagcaaaagaaaatttgccaatgcaattttaaaagtgtaagaaacttcactcatgtacctactcatgggaagaacatctaaggcaaatgaaaaattcccctccagggacataaccagctcagaaccatctgaaaaaattcatacaaaagcagaaattacccaaggcctgtgagtcctcatctcataccatgaaagccagactgtcaaaaaaagggcacatgtcactttgcaaaggaatgtattaactcctctcccagggtcaacttagtctacgtgtcttttgtataacattaatttccaccagatctactagatgttcagtcatgtcctttcaggtcctgaaggcaggctcactctctgatgcatctttttatatcatggtgggtgtgaagtgaaaagaggagacacagaaatatgcacaaacccacaattagtccatatttagaaaactttctgtgggttcaagcatttacacagagatgattttatctcatttctccattaatttcccatttgaaatgaaaaccagctaattctaaattctaaagccctgggggaaaccttccaggctttgtctatcagacagactttgtcataaaaaacacagaaaaacaaaaataaaacattacgctggaatcagcttttgagagtttgtgctttaaaaacacagtgcctaacagcaccaagcatatcatagatgctcaataaatatttgtagatttattaagagtaataacatggtgtttaaagaaccaaccaccattttgtaaaataggcaaaactacattaatttctttcacctgatttgataaagcagtgtggagcaatgaatgagagaatctgcaaattaaatatgaactctaatttgattgcagagagaaaattactgagaactttgcaaaaaacattgccacagtagccttgacactcaacagtgcaacgaagagttaatgtttccactgcaatatgaactggttcccacagctcttaggagatagagtgtaatcacttaaatgggaaatgaactctaattccacttgagaaaaggtatgttatgttcataattttatctgaaaattattaatatatttcagggagatggtcctctcattcagcatccctcaaagtaatgcaggcataagtatcaggggaccttgttatataacttcagtacagcattgtcttatacaagtgttctctcttccacatctgtagtagctgctttctaatattgtagatttttacagttgtgacacccctgggatgacagacatgagaatatggaggattaaaggttacaaaacttaaacaaaaaagggaagctcctctatgttatgtgaaaaccccttacaaaaggcagtttattgacaaataaatgctttatacattcaggtttttcccatctctcaatagtgatggtttccaaagaagaaactcagtagtgaagaatacatacttttttttttttgcattagtttgatcagttgaaaatcagaaccttcaaagcatcttgtgaatgagagaaatggaactggacctgggcaaggcatggggatggtagagatccatatgaataaatgatttagctgttgatgtggacagcaagagagttggtgggaaatgttacagcagacctgaccacgctacaaagggtctgtgaagaacacagtacaggtatcaaaacaccaaaacaaaactaaactaaaaacaagaacaaactgcaactttgccaaactgtaaacaaggtaaagcatttcacaggttcaaagttcaagggaagtaaacgtctttaaattatttttgtcagttcaaccctgatttaaaaatatggctagcaaaaacaaggaagccacagctgtcgacatcctgagcaagcatcggtctcctttgagaagctgcactcccaagcctcttctcaagctgctacacgaggaggagacacttctctcttgaattccatctcagttctctttatttccacactcttggaatacatcgattgctttccattttggtgtctacagttctggctgctatagatttagacgtggggatactggaggagggaaggcaaattctcggaggatgctccgggcaacttcgacattattctgggctatctctaaggctctcttcacctcttcaaaggcataaccctctcccatgagttttgcaatttttgcatcgacattttccaatgccgcctcaggcccatggggttttctgtggtgaatttctggtgcagtcctgcgcggtcgtggtttagggggtctggctggtgcctgtgaaccatctgaacatgaaggaagctgatcatagtcctgtgatgttctgttagttttgacattttcacctggtaaccttctagcaggaggcaaaggaacttggccacttgctagatcaacaaagggatcttggcagtcagagacggggcatctgaaggaagaagaaaaagatcctgtcctgaggatggccggctactggagccaggaggttttgaatgttcaatgagactatgccttgcaggaggtgggggaggtgggagagatggagggagggcatcaaaagcatcttcacctaatggagggatgagaagatcataatcagagggcgtcctgttgagtgaagaaccatgctttggattgtcccgagttggaggcctggcaggtggtaatggcacgggatcagaggctgaatcaaaaacatctccctttaaatatatgcttaagtcagggatgtttgatttcttctctgaagatggaccatgtgttccattcagcatacagtgaccattatcacaagaccgaacaggaggttttacattatgacaatgagatggttgtgaattcagggaaacagggtgggatgaaggaatcttgtattcatcatcatcttcctctactgggtctcttgttttctctgaaagagaatttgctaacggaccagtacactttatgctagggaggagggtggtaactggaggaggaggagaaagccggggaggaacatcatattcttcacttccaaggtgaccattggaaaagaccttagctccttctaaaggcaaatcatggcgtctgtgtttccgcataagcactgggtcagagcccactctactgtgccttccattgacatttgaactcgctgtgattccaggttttggagagccctcccctaggagtcgacatcccacaagctgattagtcccaaacacatcccgagggcaccatgcttcaagaggcattggcgggtctctggaaggcacgctttccacatgatggatgtgtctactcagtctattgtctggtgggattggtggaggtctttcaggtggcggtggaggaggatctcttaagggaggaggtggtgctgggagtggtttatcttgttttctcaccatgcaaggagaagactttggtgaacccgttgggctgccacagggagatctaactatgcctttctgaattagatccaggcgaggaggcacgggtggcaggcttagatgtgggatctggagtgggtcaggctgtggctttcttctctgggcaaggggagaggatcctggtgatgtgactggtgagttctgcctgtcagtgcactttcggacgtttgccaaccgattcatcatcaaggactcctcacgatcatcatcgtcgtccaagtctagcatcggcatgccaaaggggtcaatgatgctgcaacacctggagccttcatctcttggatcaaaggggtccacgattatgggctcagttccttttatttcacaacgacagaaagggcagccctgaccatccgactcctgccatgccgtaaggcaagaggtgcacatcaaatgcccacaaggctcaatcttgacatctttgtcattctctgcacaaatcttacagagctgaaaagtggagcccatttcacaatataattcatattgttcctgtgtaacttttatatggtcatgaggtgtaggttcacataatccagttaaatcaggattataactcctcccatcaggataaagataaaatccttccctgctgccatcaatcagggcttgaaataagggcttgttatgaggtatggtctgtaagatattcccatccccagtcacatagccaatggcccactgtcccaatcgagtgcaacttaaccggaaaatatagcttccgggtttggtgctatatttctgtagtcgtgctttaacttcatcatatgtgagaaatgccatgtaacctggatgtgtcacagctaagaaattccaattccgcaaaatagagccccaaggctgaaacagcctggtaaaaatatcaaattcaaaaactgaaatgtaatcattgcaagttaaatcaattgttgattttagagccattgcttccaggccagagctaatctggtggacctcatgaaggcactgtctgaatactttccatggtacgatagttttgtctccaaaaaactttctccagaattcagcagcatctgcttttgtgatacgaaagttatctccctggaattgaccattgggaaagattgctttgatttctgccagcatgtgactgaagataagggacagttttgtgagatttcgtcattttttttgcctttagaagatcacaatggtaattcacaaagaactgctgtcctgtgactgttcttcatacattctctccttgccttctttaaagagtcttattgcccgttttgactttttcataaggctatcaatgtagattttaaagtactcattctcactgagttgggcaagtttctggttgtcatcatatttactcaatataagtcgtaaatgctgatatgtatcaggcaaaatatcaagtatatatggtgggctatttttcaactgaagtttgggattttggcacagtcttaccactttgtccatgagcttccaagtcttctccacggtcctgcgatctgcggcagcttgcttagggggtccaactgcatcctgaatagcatcaataatacccaaaattcgaccttttcggggatttcctcctcgaccaccagggtttctgccattcattgagtttgccatctggaattttagttctttcggcgccgtagctgtccagagacacgcgtgtgcgcgggtcccactccacacgcacgcagcccagtgtgtgtggggagccccggctgggagtgggatcgctgagaacagctcgctcccgaagaaggagcaacccagcgcgcaggcctccgagacgtggaaacgcaacaattaccgtcaagacaaatccacacccgctctcccctcccgcccgactcggggaggccgcgggacgccgcagcagcactagcaggaggaggagaccgctcgctggac

SEQ ID NO: 9434 - RNA, 5759 nt, Homo sapiens
  source 1..5759: mol_type = other RNA
aggaggcatcttgagaaatggaaggaatgtctaactttttggatcacagtgaaacaaagtctggatcacttccagacatcaacgagcagtcgcttttacaataaaaaaaaatttttttaggtttaatttcataggtgatagatagcaatgggtctttcttgacagtgtttaatagaaagttttcctcttttcattccattacgtatgaatttttgattcattctttttaaatgacaatactaatggttgctattgagtacaagatgcagagattttgctggaggctggtaaattttctctgcaaaacagatatccccccaccccccacccccaaatttcaggtccaggtttgctatatcatcactagtccttttttaattctcactggaaattttcaaatattgtttataaactgaatgagaatgtgctatgttctctaacattcttattttacatcattctctaatatattaggaatgttgcaacaatgttatcacaatgaagtggcaacttttggcctttagactgtacctatcatcagcaatcataaaaaggccaaaataaacagtgctattccaaggtgacatctgaaactgttaaaacaagtgaaaaatcataatgacaaaacaggggttcataaagcaaaagaaaatttgccaatgcaattttaaaagtgtaagaaacttcactcatgtacctactcatgggaagaacatctaaggcaaatgaaaaattcccctccagggacataaccagctcagaaccatctgaaaaaattcatacaaaagcagaaattacccaaggcctgtgagtcctcatctcataccatgaaagccagactgtcaaaaaaagggcacatgtcactttgcaaaggaatgtattaactcctctcccagggtcaacttagtctacgtgtcttttgtataacattaatttccaccagatctactagatgttcagtcatgtcctttcaggtcctgaaggcaggctcactctctgatgcatctttttatatcatggtgggtgtgaagtgaaaagaggagacacagaaatatgcacaaacccacaattagtccatatttagaaaactttctgtgggttcaagcatttacacagagatgattttatctcatttctccattaatttcccatttgaaatgaaaaccagctaattctaaattctaaagccctgggggaaaccttccaggctttgtctatcagacagactttgtcataaaaaacacagaaaaacaaaaataaaacattacgctggaatcagcttttgagagtttgtgctttaaaaacacagtgcctaacagcaccaagcatatcatagatgctcaataaatatttgtagatttattaagagtaataacatggtgtttaaagaaccaaccaccattttgtaaaataggcaaaactacattaatttctttcacctgatttgataaagcagtgtggagcaatgaatgagagaatctgcaaattaaatatgaactctaatttgattgcagagagaaaattactgagaactttgcaaaaaacattgccacagtagccttgacactcaacagtgcaacgaagagttaatgtttccactgcaatatgaactggttcccacagctcttaggagatagagtgtaatcacttaaatgggaaatgaactctaattccacttgagaaaaggtatgttatgttcataattttatctgaaaattattaatatatttcagggagatggtcctctcattcagcatccctcaaagtaatgcaggcataagtatcaggggaccttgttatataacttcagtacagcattgtcttatacaagtgttctctcttccacatctgtagtagctgctttctaatattgtagatttttacagttgtgacacccctgggatgacagacatgagaatatggaggattaaaggttacaaaacttaaacaaaaaagggaagctcctctatgttatgtgaaaaccccttacaaaaggcagtttattgacaaataaatgctttatacattcaggtttttcccatctctcaatagtgatggtttccaaagaagaaactcagtagtgaagaatacatacttttttttttttgcattagtttgatcagttgaaaatcagaaccttcaaagcatcttgtgaatgagagaaatggaactggacctgggcaaggcatggggatggtagagatccatatgaataaatgatttagctgttgatgtggacagcaagagagttggtgggaaatgttacagcagacctgaccacgctacaaagggtctgtgaagaacacagtacaggtatcaaaacaccaaaacaaaactaaactaaaaacaagaacaaactgcaactttgccaaactgtaaacaaggtaaagcatttcacaggttcaaagttcaagggaagtaaacgtctttaaattatttttgtcagttcaaccctgatttaaaaatatggctagcaaaaacaaggaagccacagctgtcgacatcctgagcaagcatcggtctcctttgagaagctgcactcccaagcctcttctcaagctgctacacgaggaggagacacttctctcttgaattccatctcagttctctttatttccacactcttggaatacatcgattgctttccattttggtgtctacagttctggctgctatagatttagacgtggggatactggaggagggaaggcaaattctcggaggatgctccgggcaacttcgacattattctgggctatctctaaggctctcttcacctcttcaaaggcataaccctctcccatgagttttgcaatttttgcatcgacattttccaatgccgcctcaggcccatggggttttctgtggtgaatttctggtgcagtcctgcgcggtcgtggtttagggggtctggctggtgcctgtgaaccatctgaacatgaaggaagctgatcatagtcctgtgatgttctgttagttttgacattttcacctggtaaccttctagcaggaggcaaaggaacttggccacttgctagatcaacaaagggatcttggcagtcagagacggggcatctgaaggaagaagaaaaagatcctgtcctgaggatggccggctactggagccaggaggttttgaatgttcaatgagactatgccttgcaggaggtgggggaggtgggagagatggagggagggcatcaaaagcatcttcacctaatggagggatgagaagatcataatcagagggcgtcctgttgagtgaagaaccatgctttggattgtcccgagttggaggcctggcaggtggtaatggcacgggatcagaggctgaatcaaaaacatctccctttaaatatatgcttaagtcagggatgtttgatttcttctctgaagatggaccatgtgttccattcagcatacagtgaccattatcacaagaccgaacaggaggttttacattatgacaatgagatggttgtgaattcagggaaacagggtgggatgaaggaatcttgtattcatcatcatcttcctctactgggtctcttgttttctctgaaagagaatttgctaacggaccagtacactttatgctagggaggagggtggtaactggaggaggaggagaaagccggggaggaacatcatattcttcacttccaaggtgaccattggaaaagaccttagctccttctaaaggcaaatcatggcgtctgtgtttccgcataagcactgggtcagagcccactctactgtgccttccattgacatttgaactcgctgtgattccaggttttggagagccctcccctaggagtcgacatcccacaagctgattagtcccaaacacatcccgagggcaccatgcttcaagaggcattggcgggtctctggaaggcacgctttccacatgatggatgtgtctactcagtctattgtctggtgggattggtggaggtctttcaggtggcggtggaggaggatctcttaagggaggaggtggtgctgggagtggtttatcttgttttctcaccatgcaaggagaagactttggtgaacccgttgggctgccacagggagatctaactatgcctttctgaattagatccaggcgaggaggcacgggtggcaggcttagatgtgggatctggagtgggtcaggctgtggctttcttctctgggcaaggggagaggatcctggtgatgtgactggtgagttctgcctgtcagtgcactttcggacgtttgccaaccgattcatcatcaaggactcctcacgatcatcatcgtcgtccaagtctagcatcggcatgccaaaggggtcaatgatgctgcaacacctggagccttcatctcttggatcaaaggggtccacgattatgggctcagttccttttatttcacaacgacagaaagggcagccctgaccatccgactcctgccatgccgtaaggcaagaggtgcacatcaaatgcccacaaggctcaatcttgacatctttgtcattctctgcacaaatcttacagagctgaaaagtggagcccatttcacaatataattcatattgttcctgtgtaacttttatatggtcatgaggtgtaggttcacataatccagttaaatcaggattataactcctcccatcaggataaagataaaatccttccctgctgccatcaatcagggcttgaaataagggcttgttatgaggtatggtctgtaagatattcccatccccagtcacatagccaatggcccactgtcccaatcgagtgcaacttaaccggaaaatatagcttccgggtttggtgctatatttctgtagtcgtgctttaacttcatcatatgtgagaaatgccatgtaacctggatgtgtcacagctaagaaattccaattccgcaaaatagagccccaaggctgaaacagcctggtaaaaatatcaaattcaaaaactgaaatgtaatcattgcaagttaaatcaattgttgattttagagccattgcttccaggccagagctaatctggtggacctcatgaaggcactgtctgaatactttccatggtacgatagttttgtctccaaaaaactttctccagaattcagcagcatctgcttttgtgatacgaaagttatctccctggaattgaccattgggaaagattgctttgatttctgccagcatgtgactgaagataagggacagttttgtgagatttcgtctgtcctgtgactgttcttcatacattctctccttgccttctttaaagagtcttattgcccgttttgactttttcataaggctatcaatgtagattttaaagtactcattctcactgagttgggcaagtttctggttgtcatcatatttactcaatataagtcgtaaatgctgatatgtatcaggcaaaatatcaagtatatatggtgggctatttttcaactgaagtttgggattttggcacagtcttaccactttgtccatgagcttccaagtcttctccacggtcctgcgatctgcggcagcttgcttagggggtccaactgcatcctgaatagcatcaataatacccaaaattcgaccttttcggggatttcctcctcgaccaccagggtttctgccattcattgagtttgccatctggaattttagttcgtcaagacaaatccacacccgctctcccctcccgcccgactcggggaggccgcgggacgccgcagcagcactagcaggaggaggagaccgctcgctggac

SEQ ID NO: 9435 - RNA, 5911 nt, Homo sapiens
  source 1..5911: mol_type = other RNA
aggaggcatcttgagaaatggaaggaatgtctaactttttggatcacagtgaaacaaagtctggatcacttccagacatcaacgagcagtcgcttttacaataaaaaaaaatttttttaggtttaatttcataggtgatagatagcaatgggtctttcttgacagtgtttaatagaaagttttcctcttttcattccattacgtatgaatttttgattcattctttttaaatgacaatactaatggttgctattgagtacaagatgcagagattttgctggaggctggtaaattttctctgcaaaacagatatccccccaccccccacccccaaatttcaggtccaggtttgctatatcatcactagtccttttttaattctcactggaaattttcaaatattgtttataaactgaatgagaatgtgctatgttctctaacattcttattttacatcattctctaatatattaggaatgttgcaacaatgttatcacaatgaagtggcaacttttggcctttagactgtacctatcatcagcaatcataaaaaggccaaaataaacagtgctattccaaggtgacatctgaaactgttaaaacaagtgaaaaatcataatgacaaaacaggggttcataaagcaaaagaaaatttgccaatgcaattttaaaagtgtaagaaacttcactcatgtacctactcatgggaagaacatctaaggcaaatgaaaaattcccctccagggacataaccagctcagaaccatctgaaaaaattcatacaaaagcagaaattacccaaggcctgtgagtcctcatctcataccatgaaagccagactgtcaaaaaaagggcacatgtcactttgcaaaggaatgtattaactcctctcccagggtcaacttagtctacgtgtcttttgtataacattaatttccaccagatctactagatgttcagtcatgtcctttcaggtcctgaaggcaggctcactctctgatgcatctttttatatcatggtgggtgtgaagtgaaaagaggagacacagaaatatgcacaaacccacaattagtccatatttagaaaactttctgtgggttcaagcatttacacagagatgattttatctcatttctccattaatttcccatttgaaatgaaaaccagctaattctaaattctaaagccctgggggaaaccttccaggctttgtctatcagacagactttgtcataaaaaacacagaaaaacaaaaataaaacattacgctggaatcagcttttgagagtttgtgctttaaaaacacagtgcctaacagcaccaagcatatcatagatgctcaataaatatttgtagatttattaagagtaataacatggtgtttaaagaaccaaccaccattttgtaaaataggcaaaactacattaatttctttcacctgatttgataaagcagtgtggagcaatgaatgagagaatctgcaaattaaatatgaactctaatttgattgcagagagaaaattactgagaactttgcaaaaaacattgccacagtagccttgacactcaacagtgcaacgaagagttaatgtttccactgcaatatgaactggttcccacagctcttaggagatagagtgtaatcacttaaatgggaaatgaactctaattccacttgagaaaaggtatgttatgttcataattttatctgaaaattattaatatatttcagggagatggtcctctcattcagcatccctcaaagtaatgcaggcataagtatcaggggaccttgttatataacttcagtacagcattgtcttatacaagtgttctctcttccacatctgtagtagctgctttctaatattgtagatttttacagttgtgacacccctgggatgacagacatgagaatatggaggattaaaggttacaaaacttaaacaaaaaagggaagctcctctatgttatgtgaaaaccccttacaaaaggcagtttattgacaaataaatgctttatacattcaggtttttcccatctctcaatagtgatggtttccaaagaagaaactcagtagtgaagaatacatacttttttttttttgcattagtttgatcagttgaaaatcagaaccttcaaagcatcttgtgaatgagagaaatggaactggacctgggcaaggcatggggatggtagagatccatatgaataaatgatttagctgttgatgtggacagcaagagagttggtgggaaatgttacagcagacctgaccacgctacaaagggtctgtgaagaacacagtacaggtatcaaaacaccaaaacaaaactaaactaaaaacaagaacaaactgcaactttgccaaactgtaaacaaggtaaagcatttcacaggttcaaagttcaagggaagtaaacgtctttaaattatttttgtcagttcaaccctgatttaaaaatatggctagcaaaaacaaggaagccacagctgtcgacatcctgagcaagcatcggtctcctttgagaagctgcactcccaagcctcttctcaagctgctacacgaggaggagacacttctctcttgaattccatctcagttctctttatttccacactcttggaatacatcgattgctttccattttggtgtctacagttctggctgctatagatttagacgtggggatactggaggagggaaggcaaattctcggaggatgctccgggcaacttcgacattattctgggctatctctaaggctctcttcacctcttcaaaggcataaccctctcccatgagttttgcaatttttgcatcgacattttccaatgccgcctcaggcccatggggttttctgtggtgaatttctggtgcagtcctgcgcggtcgtggtttagggggtctggctggtgcctgtgaaccatctgaacatgaaggaagctgatcatagtcctgtgatgttctgttagttttgacattttcacctggtaaccttctagcaggaggcaaaggaacttggccacttgctagatcaacaaagggatcttggcagtcagagacggggcatctgaaggaagaagaaaaagatcctgtcctgaggatggccggctactggagccaggaggttttgaatgttcaatgagactatgccttgcaggaggtgggggaggtgggagagatggagggagggcatcaaaagcatcttcacctaatggagggatgagaagatcataatcagagggcgtcctgttgagtgaagaaccatgctttggattgtcccgagttggaggcctggcaggtggtaatggcacgggatcagaggctgaatcaaaaacatctccctttaaatatatgcttaagtcagggatgtttgatttcttctctgaagatggaccatgtgttccattcagcatacagtgaccattatcacaagaccgaacaggaggttttacattatgacaatgagatggttgtgaattcagggaaacagggtgggatgaaggaatcttgtattcatcatcatcttcctctactgggtctcttgttttctctgaaagagaatttgctaacggaccagtacactttatgctagggaggagggtggtaactggaggaggaggagaaagccggggaggaacatcatattcttcacttccaaggtgaccattggaaaagaccttagctccttctaaaggcaaatcatggcgtctgtgtttccgcataagcactgggtcagagcccactctactgtgccttccattgacatttgaactcgctgtgattccaggttttggagagccctcccctaggagtcgacatcccacaagctgattagtcccaaacacatcccgagggcaccatgcttcaagaggcattggcgggtctctggaaggcacgctttccacatgatggatgtgtctactcagtctattgtctggtgggattggtggaggtctttcaggtggcggtggaggaggatctcttaagggaggaggtggtgctgggagtggtttatcttgttttctcaccatgcaaggagaagactttggtgaacccgttgggctgccacagggagatctaactatgcctttctgaattagatccaggcgaggaggcacgggtggcaggcttagatgtgggatctggagtgggtcaggctgtggctttcttctctgggcaaggggagaggatcctggtgatgtgactggtgagttctgcctgtcagtgcactttcggacgtttgccaaccgattcatcatcaaggactcctcacgatcatcatcgtcgtccaagtctagcatcggcatgccaaaggggtcaatgatgctgcaacacctggagccttcatctcttggatcaaaggggtccacgattatgggctcagttccttttatttcacaacgacagaaagggcagccctgaccatccgactcctgccatgccgtaaggcaagaggtgcacatcaaatgcccacaaggctcaatcttgacatctttgtcattctctgcacaaatcttacagagctgaaaagtggagcccatttcacaatataattcatattgttcctgtgtaacttttatatggtcatgaggtgtaggttcacataatccagttaaatcaggattataactcctcccatcaggataaagataaaatccttccctgctgccatcaatcagggcttgaaataagggcttgttatgaggtatggtctgtaagatattcccatccccagtcacatagccaatggcccactgtcccaatcgagtgcaacttaaccggaaaatatagcttccgggtttggtgctatatttctgtagtcgtgctttaacttcatcatatgtgagaaatgccatgtaacctggatgtgtcacagctaagaaattccaattccgcaaaatagagccccaaggctgaaacagcctggtaaaaatatcaaattcaaaaactgaaatgtaatcattgcaagttaaatcaattgttgattttagagccattgcttccaggccagagctaatctggtggacctcatgaaggcactgtctgaatactttccatggtacgatagttttgtctccaaaaaactttctccagaattcagcagcatctgcttttgtgatacgaaagttatctccctggaattgaccattgggaaagattgctttgatttctgccagcatgtgactgaagataagggacagttttgtgagatttcgtctgtcctgtgactgttcttcatacattctctccttgccttctttaaagagtcttattgcccgttttgactttttcataaggctatcaatgtagattttaaagtactcattctcactgagttgggcaagtttctggttgtcatcatatttactcaatataagtcgtaaatgctgatatgtatcaggcaaaatatcaagtatatatggtgggctatttttcaactgaagtttgggattttggcacagtcttaccactttgtccatgagcttccaagtcttctccacggtcctgcgatctgcggcagcttgcttagggggtccaactgcatcctgaatagcatcaataatacccaaaattcgaccttttcggggatttcctcctcgaccaccagggtttctgccattcattgagtttgccatctggaattttagttctttctttaaatcaacgcggtgagtcgttattcccaagaaccaaatgaaattaacacacaaatagcccatttgaaaagagaaaagagaaaaatgacaagagcggccacggaaaggaggagttcacttctctggctcctcgcctctgccctcaacccaaagctttgtttcaggacgcctgtgtcccttccctgctcaggccccttcccggcccctcgggtctgagctgcaggaggaaggtggactgggagggga

SEQ ID NO: 9436 - RNA, 5849 nt, Homo sapiens
  source 1..5849: mol_type = other RNA
aggaggcatcttgagaaatggaaggaatgtctaactttttggatcacagtgaaacaaagtctggatcacttccagacatcaacgagcagtcgcttttacaataaaaaaaaatttttttaggtttaatttcataggtgatagatagcaatgggtctttcttgacagtgtttaatagaaagttttcctcttttcattccattacgtatgaatttttgattcattctttttaaatgacaatactaatggttgctattgagtacaagatgcagagattttgctggaggctggtaaattttctctgcaaaacagatatccccccaccccccacccccaaatttcaggtccaggtttgctatatcatcactagtccttttttaattctcactggaaattttcaaatattgtttataaactgaatgagaatgtgctatgttctctaacattcttattttacatcattctctaatatattaggaatgttgcaacaatgttatcacaatgaagtggcaacttttggcctttagactgtacctatcatcagcaatcataaaaaggccaaaataaacagtgctattccaaggtgacatctgaaactgttaaaacaagtgaaaaatcataatgacaaaacaggggttcataaagcaaaagaaaatttgccaatgcaattttaaaagtgtaagaaacttcactcatgtacctactcatgggaagaacatctaaggcaaatgaaaaattcccctccagggacataaccagctcagaaccatctgaaaaaattcatacaaaagcagaaattacccaaggcctgtgagtcctcatctcataccatgaaagccagactgtcaaaaaaagggcacatgtcactttgcaaaggaatgtattaactcctctcccagggtcaacttagtctacgtgtcttttgtataacattaatttccaccagatctactagatgttcagtcatgtcctttcaggtcctgaaggcaggctcactctctgatgcatctttttatatcatggtgggtgtgaagtgaaaagaggagacacagaaatatgcacaaacccacaattagtccatatttagaaaactttctgtgggttcaagcatttacacagagatgattttatctcatttctccattaatttcccatttgaaatgaaaaccagctaattctaaattctaaagccctgggggaaaccttccaggctttgtctatcagacagactttgtcataaaaaacacagaaaaacaaaaataaaacattacgctggaatcagcttttgagagtttgtgctttaaaaacacagtgcctaacagcaccaagcatatcatagatgctcaataaatatttgtagatttattaagagtaataacatggtgtttaaagaaccaaccaccattttgtaaaataggcaaaactacattaatttctttcacctgatttgataaagcagtgtggagcaatgaatgagagaatctgcaaattaaatatgaactctaatttgattgcagagagaaaattactgagaactttgcaaaaaacattgccacagtagccttgacactcaacagtgcaacgaagagttaatgtttccactgcaatatgaactggttcccacagctcttaggagatagagtgtaatcacttaaatgggaaatgaactctaattccacttgagaaaaggtatgttatgttcataattttatctgaaaattattaatatatttcagggagatggtcctctcattcagcatccctcaaagtaatgcaggcataagtatcaggggaccttgttatataacttcagtacagcattgtcttatacaagtgttctctcttccacatctgtagtagctgctttctaatattgtagatttttacagttgtgacacccctgggatgacagacatgagaatatggaggattaaaggttacaaaacttaaacaaaaaagggaagctcctctatgttatgtgaaaaccccttacaaaaggcagtttattgacaaataaatgctttatacattcaggtttttcccatctctcaatagtgatggtttccaaagaagaaactcagtagtgaagaatacatacttttttttttttgcattagtttgatcagttgaaaatcagaaccttcaaagcatcttgtgaatgagagaaatggaactggacctgggcaaggcatggggatggtagagatccatatgaataaatgatttagctgttgatgtggacagcaagagagttggtgggaaatgttacagcagacctgaccacgctacaaagggtctgtgaagaacacagtacaggtatcaaaacaccaaaacaaaactaaactaaaaacaagaacaaactgcaactttgccaaactgtaaacaaggtaaagcatttcacaggttcaaagttcaagggaagtaaacgtctttaaattatttttgtcagttcaaccctgatttaaaaatatggctagcaaaaacaaggaagccacagctgtcgacatcctgagcaagcatcggtctcctttgagaagctgcactcccaagcctcttctcaagctgctacacgaggaggagacacttctctcttgaattccatctcagttctctttatttccacactcttggaatacatcgattgctttccattttggtgtctacagttctggctgctatagatttagacgtggggatactggaggagggaaggcaaattctcggaggatgctccgggcaacttcgacattattctgggctatctctaaggctctcttcacctcttcaaaggcataaccctctcccatgagttttgcaatttttgcatcgacattttccaatgccgcctcaggcccatggggttttctgtggtgaatttctggtgcagtcctgcgcggtcgtggtttagggggtctggctggtgcctgtgaaccatctgaacatgaaggaagctgatcatagtcctgtgatgttctgttagttttgacattttcacctggtaaccttctagcaggaggcaaaggaacttggccacttgctagatcaacaaagggatcttggcagtcagagacggggcatctgcttatggttctgttttgaatcattatcatgttctatcttgcatcatatcctaagtttgctatttgtcagccatagggtaaactgggctctctaaagcaaattataaagttggaagcattcaggctgaaggaagaagaaaaagatcctgtcctgaggatggccggctactggagccaggaggttttgaatgttcaatgagactatgccttgcaggaggtgggggaggtgggagagatggagggagggcatcaaaagcatcttcacctaatggagggatgagaagatcataatcagagggcgtcctgttgagtgaagaaccatgctttggattgtcccgagttggaggcctggcaggtggtaatggcacgggatcagaggctgaatcaaaaacatctccctttaaatatatgcttaagtcagggatgtttgatttcttctctgaagatggaccatgtgttccattcagcatacagtgaccattatcacaagaccgaacaggaggttttacattatgacaatgagatggttgtgaattcagggaaacagggtgggatgaaggaatcttgtattcatcatcatcttcctctactgggtctcttgttttctctgaaagagaatttgctaacggaccagtacactttatgctagggaggagggtggtaactggaggaggaggagaaagccggggaggaacatcatattcttcacttccaaggtgaccattggaaaagaccttagctccttctaaaggcaaatcatggcgtctgtgtttccgcataagcactgggtcagagcccactctactgtgccttccattgacatttgaactcgctgtgattccaggttttggagagccctcccctaggagtcgacatcccacaagctgattagtcccaaacacatcccgagggcaccatgcttcaagaggcattggcgggtctctggaaggcacgctttccacatgatggatgtgtctactcagtctattgtctggtgggattggtggaggtctttcaggtggcggtggaggaggatctcttaagggaggaggtggtgctgggagtggtttatcttgttttctcaccatgcaaggagaagactttggtgaacccgttgggctgccacagggagatctaactatgcctttctgaattagatccaggcgaggaggcacgggtggcaggcttagatgtgggatctggagtgggtcaggctgtggctttcttctctgggcaaggggagaggatcctggtgatgtgactggtgagttctgcctgtcagtgcactttcggacgtttgccaaccgattcatcatcaaggactcctcacgatcatcatcgtcgtccaagtctagcatcggcatgccaaaggggtcaatgatgctgcaacacctggagccttcatctcttggatcaaaggggtccacgattatgggctcagttccttttatttcacaacgacagaaagggcagccctgaccatccgactcctgccatgccgtaaggcaagaggtgcacatcaaatgcccacaaggctcaatcttgacatctttgtcattctctgcacaaatcttacagagctgaaaagtggagcccatttcacaatataattcatattgttcctgtgtaacttttatatggtcatgaggtgtaggttcacataatccagttaaatcaggattataactcctcccatcaggataaagataaaatccttccctgctgccatcaatcagggcttgaaataagggcttgttatgaggtatggtctgtaagatattcccatccccagtcacatagccaatggcccactgtcccaatcgagtgcaacttaaccggaaaatatagcttccgggtttggtgctatatttctgtagtcgtgctttaacttcatcatatgtgagaaatgccatgtaacctggatgtgtcacagctaagaaattccaattccgcaaaatagagccccaaggctgaaacagcctggtaaaaatatcaaattcaaaaactgaaatgtaatcattgcaagttaaatcaattgttgattttagagccattgcttccaggccagagctaatctggtggacctcatgaaggcactgtctgaatactttccatggtacgatagttttgtctccaaaaaactttctccagaattcagcagcatctgcttttgtgatacgaaagttatctccctggaattgaccattgggaaagattgctttgatttctgccagcatgtgactgaagataagggacagttttgtgagatttcgtctgtcctgtgactgttcttcatacattctctccttgccttctttaaagagtcttattgcccgttttgactttttcataaggctatcaatgtagattttaaagtactcattctcactgagttgggcaagtttctggttgtcatcatatttactcaatataagtcgtaaatgctgatatgtatcaggcaaaatatcaagtatatatggtgggctatttttcaactgaagtttgggattttggcacagtcttaccactttgtccatgagcttccaagtcttctccacggtcctgcgatctgcggcagcttgcttagggggtccaactgcatcctgaatagcatcaataatacccaaaattcgaccttttcggggatttcctcctcgaccaccagggtttctgccattcattgagtttgccatctggaattttagttcaataaggggtggcaggtgggcgtgagcgtcgggaccgggagccaaagccatctggggctgaaag

SEQ ID NO: 9437 - RNA, 931 nt, Homo sapiens
  source 1..931: mol_type = other RNA
aggagggaaggggctgagaacaggaggaacactaggaggaaaagggtgacccaggagggaagagttcgggacactgcagagctggtttggagacatcctctcaccatagggagcaggataacgaggtggcattgggggccgaacatggacaggcttcggacacagaatctgttgggtgaagctgggtacagccatctgtttaggtggggtgcctatggggacagctctaacaggaggactgccaatgataggtgaagttgaccgccttggtaatgctcgttcagaaaggtcccgatcatcttctggaccctgggggggcctctgaggcaaagcatattctaatacagacactgtaggcatttcctgagcaagcagtggtcctcggattcgcctcagaacttcagatccatcccagatactggaattcagacttcctggttggggttgtaaaactggcctggtctgcactgccctcataatagctggatcttctagttcattttcaatcaccatcttactgagcctttctgccagattctcctcatggtcacccaacaagtccatttcatctctctctccattgcctgtttgttcattaactgccactggtagcttttcttccaattcagccaggcgctcatgtgcttcctgccaatcatcatcaactgcacctgacccaaatgtatcatcattgaattgatcaatctcttcatcttcttctcccagtccctgaaatgcatcttcatcttcatccagaggacaatcctccaaagactcgtagcggaacattcttggggaggggggcagggagcggggaggggagagggggagggagggaagaagcgctgactccccggctcctccgcgcgcgggtcctccaccggctcgcgacccctggccgccgccgtacgccggagcgtgcgtggggacg

SEQ ID NO: 9438 - RNA, 227 nt, Homo sapiens
  source 1..227: mol_type = other RNA
aggagggaggagatgggccaagttggtccaggtgccatccgttgctggggaagggccataggtgaaggcatccagtgcactgccattgccggctgagaaccagatggggcctgttgtggcagcctctggtgaggaagggaaggaaacaggacctgtgggtagggctggacacccaagggccaggagaagtagcagccatgtaccggccatggcccactcggaaggag

SEQ ID NO: 9439 - RNA, 398 nt, Homo sapiens
  source 1..398: mol_type = other RNA
aggagggaggagatgggccaagttggtccaggtgccatccgttgctggggaagggccataggtgaaggcatccagtgcactgccattgccggctgagaaccagatggggctgtcaaggccagggggtgcaacatcaaggaccaggcagaccaccaccatctgctgctttccatccaccagcagcatgattggtggggccagagaaggaaagggtgtgccgcccacaccctgttgtggcagcctctggtgaggaagggaaggaaacaggacctgtgggtagggctggacacccaagggccaggagaagtagcagccatgtaccggccatggcccactcggaaggaggcaggacccagctgcagacctgagttgcggctgggggaggaggcacccacaag

SEQ ID NO: 9440 - RNA, 302 nt, Homo sapiens
  source 1..302: mol_type = other RNA
aggagggaggagatgggccaagttggtccaggtgccatccgttgctggggaagggccataggtgaaggcatccagtgcactgccattgccggctgagaaccagatggggctgtcaaggccagggggtgcaacatcaaggaccaggcagaccaccaccatctgctgctttccatccaccagcagcatgattggtggggccagagaaggaaagggtgtgccgcccacacctgtgggtagggctggacacccaagggccaggagaagtagcagccatgtaccggccatggcccactcggaaggag

SEQ ID NO: 9441 - RNA, 334 nt, Homo sapiens
  source 1..334: mol_type = other RNA
aggagggaggagatgggccaagttggtccaggtgccatccgttgctggggaagggccataggtgaaggcatccagtgcactgccattgccggctgagaaccagatggggctgtcaaggccagggggtgcaacatcaaggaccaggcagaccaccaccatctgctgctttccatccaccagcagcatgattggtggggccagagaaggaaagggtgtgccgcccacacctgtttatccatcctttcttctatcagccatctatcctccatgtattctttctttcttttttttttttttgagatggaattttgctctgttgcccaggctagagtgc

SEQ ID NO: 9442 - RNA, 636 nt, Homo sapiens
  source 1..636: mol_type = other RNA
aggagggaggagatgggccaagttggtccaggtgccatccgttgctggggaagggccataggtgaaggcatccagtgcactgccattgccggctgagaaccagatggggctgtgggtagggctggacacccaagggccaggagaagtagcagccatgtaccggccatggcccactcggaaggaggcaggacccagctgcagacctgagttgcggctgggggaggaggcacccacaagactgccttctaggccacaggcccagctgcacctcagctgctctaccacgagccgtttcccctggtgacgggcccctactcctgccctggcccccaaacccaatcttgtctcacgggccagggagcacagggtgcctctcccacaccaggagccggacacctgcactccctctgaagagacagcacttcagtctgcaaagtcccgcttcagggcagctaccatccacaggacacggagcaccaggtggcttgacaggggcttgacatacagcccttcacttgatccactcaaccactgagttacatttcacaggtgaggcaactgaggctcacagagagtgagggacccgcccagggccacacagctgacaggtaccagagccagggcttgaactgtttt

SEQ ID NO: 9443 - RNA, 640 nt, Homo sapiens
  source 1..640: mol_type = other RNA
aggagggaggagatgggccaagttggtccaggtgccatccgttgctggggaagggccataggtgaaggcatccagtgcactgccattgccggctgagaaccagatggggctgtgggtagggctggacacccaagggccaggagaagtagcagccatgtaccggccatggcccactcggaaggaggcaggacccagctgcagacctgagttgcggctgggggaggaggcacccacaagactgccttctaggccacaggcccagctgcacctcagctgctctaccacgagccgtttcccctggtgacgggcccctactcctgccctggcccccaaacccaatcttgtctcacgggccagggagcacagggtgcctctcccacaccaggagccggacacctgcactccctctgaagagacagcacttcagtctgcaaagtcccgcttcagggcagctaccatccacaggacacggagcaccaggtggcttgacaggggcttgacatacagcccttcacttgatccactcaaccactgagttacatttcacaggtgaggcaactgaggctcacagagagtgagggacccgcccagggccacacagctgacaggtaccagagccagggcttgaactgtttttaga

SEQ ID NO: 9444 - RNA, 3043 nt, Homo sapiens
  source 1..3043: mol_type = other RNA
aggcaagatgctggcatagctctcaaaatgctcgcacaagggacactccatggcaggtccctgcagcagagcaaagtcacaacatttgaggttctctgcactctgaggcctacagagctcggctggccgagtgaggctgggaggatggtgcccgctggtcagggcagctgagtggggctgggaggatggtgcccgctggtcagggcagccctctgggtcagggtgactgagcaaggctggaaggatggtgcctgctggtcagggtggccgcgtgaggctgggagggtggtgcccgctggtccgggtggccaagagaggctggaaggatggtgtctgctggtcagggcggcccaggaggtgctgtccaggcggagcccggggctggtgtgggtgcgccatgctcctgagaagtttctgggttgtggctttaatgttctcctgcaataagaacgctgacacttggctgaaaggtcctcacgtctcccccagtacacttctgagatgccaggaaggcattctgaacatcaggctgattcctgggactcccctccagggtgacctcaccggagtcaggagcccccgccccgcgcccactgccccactaggatggctctgcagtggcctgaggacagtgaacactggggtgtaaagttgcccactgtgatggttttgacctttgaagaaatttgggaaccaagtgaaagcccggcagctatttctaggcatttcagagggtgcttccctgcacgatttcagagggtgcttccctgcacgatttcagaaggtgcttccctgcacgacttcacagggtgcttccctgcacgatttcagagggtgcttccctgcacgatttcagagggtgcttccctgcacgacttcacagggtgcttccctgcacgatttcacagggtgcttccctgcacgatttcacagggtgcttccctgcacgatttcagaggctgcttccctgcacgcactctgccgcacaccgcactccctgggccaggagcctgctgcacagaaggaggttccttttcttctctttccagcgcttttcttctccttttcttcatctctgctcctcctctaactgaggaatgtgcgaatcttttttgttagttttgaggctgcttcttatgcatatttcatctggaacttcttgctttgggggtgatctgctctaccagcctgaatgctgggctggtctgtggggctggggcccaccgcccacgtcggaaggccgaggggcagatgcaggctggaccgaagctgccgagggcaccccaggggccccactgcatggctgggacgggaagctcagcaggtggtggtgtccaaggtcctgaggaacctttgtcccaagtccatccaggtaagtcaggccgcctctctgggaggaaggctgggccaagagggcacgtggtgtggcccagttccggggacgggggtctgagctcagggactggcactccagcaggaggagagaagccagaggaccaagcacagttggggcacagaggccgggcagggacaagcggccccgggcactgaagctggctgggcagggatgagtggtcccagggctcgctgcagagctcggggacccagagggcagagagtccagactggggccttcagcggcagatgaaaggcttaagcagagtggacatcacaggcaggcagcagcgggaagtgctgggctgcccactacaccaggagcctctcctgctgggtgctctgaggtgacccaaacacgtccaatggatggcagtgaatactccctggtctctggtgctgagccccgttcgccatcgggaacttggaaaatgctctgtggctgcaaggagcctctggtggcttctccatcactgcggtgtcttgatcagagagactctctgcagtggaaaggtctctccctcgctggcacgttcccacatctgactgggctgcttttccgggggtccccagggcacggaacacagtgcgcacggccctgcgcccccatcagacgcgggacacgagggagccacggagcaggtgtccggcgaggctcgcaccgcagggcccgagtccgcagatggccccggctcagggcttcttccgagggtggcgtttctgatggcggatgagacaggagctgtaggcaaaggctttcccacagtgcgtgcattcgtagggcttctccccggtgtgcgtcttctgatgtttcaggagattggagccgcagttaaaggctttcccgcactccccgcatttgaagggcttctctcccgtgtgagtcctctggtgtttggtgacgtcagagctgtgccggaaggccttcccgcactgcgcacacttgaagggcttctctccagtgtggaccctctgatggcgaatgtggtctgtcttgtgcttaaagatccgcccacactcactgcactcatagggtttcttcctctgaaaaggaatgaacacgggaaccccctcaaagtcatctttaaatgaagcgtcgaaggcatcaaagacgtgctcttcgtcttcaggactcaggcagggctctgtgcggggcttcctgggcacagtgggcctctcaggtggctttctgtccccggacaccttctcctctctgagcgcactcttctgcacgtctgcctcctcccttggggtcggcgtcttcttttttctgcctgcaggcttctccatcattctgttccttggaagcgtgagggctaaggggctgctgacctctctgttggccccacttcctcaatggcttgcttcccacgcacctctccacactcccagcgtgggactgatgctctgcaccaggaggccaagggccaccatcctcttggtgctggctggagacgagaggcgacgaggacctcccgctgcagagcgcggacgcgcccgggccctaccaggactgctggagggcggggagaggcgcgcgcccctcgcgggggccggaggcaggaaaggagagccctagatgcgggaccccccaacagctccccaccagtgccagcgtccccgtcggccctaggcaccggcaggaaat

SEQ ID NO: 9445 - RNA, 69 nt, Homo sapiens
  source 1..69: mol_type = other RNA
aggcatgggaggtcaggtgagctcagctccctgcctcacctgagctcccgtgcctgtgcaccctctatt

SEQ ID NO: 9446 - RNA, 68 nt, Homo sapiens
  source 1..68: mol_type = other RNA
aggccatcagcagtccaatgaagacattgggtcttcatgtcttcattggactgctgatggcctgtcat

SEQ ID NO: 9447 - RNA, 55 nt, Homo sapiens
  source 1..55: mol_type = other RNA
aggcctgtggctcctccctcaggactgcttcctatccatgacggtctcctggtac

SEQ ID NO: 9448 - RNA, 103 nt, Homo sapiens
  source 1..103: mol_type = other RNA
aggcctgtggctcctccctcagtaatgtgggtggatactgcccctggctggtgaccaggccgagcccgtggtggctgccatcttgcgtcgctcttgcttgaag

SEQ ID NO: 9449 - RNA, 41 nt, Homo sapiens
  source 1..41: mol_type = other RNA
aggcggggcgccgcgggaccgcacgccggcttgcgcgagac

SEQ ID NO: 9450 - RNA, 104 nt, Homo sapiens
  source 1..104: mol_type = other RNA
aggcggggcgccgcgggaccgcacgccggcttgcgcgagaccacgctccctcaccgcgcgggcaataagtcccgccccgcacaggccacgccctccgcgcacag

SEQ ID NO: 9451 - RNA, 2094 nt, Homo sapiens
  source 1..2094: mol_type = other RNA
aggcggggcgccgcgggaccgccctcgtgtctgtggcggtgggatcccgcggccgtgttttcctggtggcccggccgtgcctgaggtttctccccgagccgccgcctctgcgggctcccgggtgcccttgccctcgcggtccccggccctcgcccgtctgtgccctcttccccgcccgccgcccgccgatcctcttcttccccccgagcggctcaccggcttcacgtccgttggtggccccgcctgggaccgaacccggcaccgcctcgtggggcgccgccgccggccactgatcggcccggcgtccgcgtcccccggcgcgcgccttggggaccgggtcggtggcgccccgcgtggggcccggtgggcttcccggagggttccgggggtcggcctgcggcgcgtgcgggggaggagacggttccgggggaccggccgcgactgcggcggcggtggtgggggcagccgcggggatcgccgagggccggtcggccgccccgggtgccgcgcggtgccgccggcggcggtgaggccccgcgcgtgtgtcccggccgcggtcggccgcgctcgaggggtccccgtggcgtccccttccccgccggccgcctttctcgcgccttccccgtcgccccggcctcgcccgtggtctctcgtcttctcccggcccgctcttccgaaccgggtcggcgcgtcccccgggtgcgcctcgcttcccgggcctgccgcggcccttccccgaggcgtccgtcccgggcgtcggcgtcggggagagcccgtcctccccgcgtggcgtcgccccgttcggcgcgcgcgtgcgcccgagcgcggcccggtggtccctgccggacaggcgttcgtgcgacgtgtggcgtgggtcgacctccgccttgccggtcgctcgccctttccccgggtcggggggtggggcccgggccggggcctcggccccggtcgcggtcccccgtcccgggcgggggcgggcgcgccggccggcctcggtcggccctcccttggccgtcgtgtggcgtgtgccacccctgcgcccgcgcccgccggcggggctcggagccgggcttcggccgggccccgggccctcgaccggaccggtgcgcgggcgctgcggccgcacggcgcgactgtccccgggccgggcaccgcggtccgcctctcgctcgccgcccggacgtcggggccgccccgcggggcgggcggagcgccgtccccgcctcgccgccgcccgcgggcgccggccgcgcgcgcgcgcgcgtggccgccggtccctcccggccgccgggcgcgggtcgggccgtccgcctcctcgcgggcgggcgcgacgaagaagcgtcgcgggtctgtggcgcggggccccggtggtcgtgtcgcgtggggggcgggtggttggggcgtccggttcgccgcgccccgccccggccccaccggtcccggccgccgcccccgcgcccgctcgctccctcccgtccgcccgtccgcggcccgtccgtccgtccgtcgtcctcctcgcttgcggggcgccgggcccgtcctcgcgaggccccccggccggccgtccggccgcgtcggggcctcgccgcgctctaccttacctacctggttgatcggttctcggcggcgtcgcggcgggtctgggggggtctcggtgccctcctccccgccggggcccgtcgtccggccccgccgcgccggctccccgtcttcggggccggccggattcccgtcgcctccgccgcgccgctccgcgccgccgggcacggccccgctcgctctccccggccttcccgctagggcgtctcgagggtcgggggccggacgccggtcccctcccccgcctcctcgtccgcccccccgccgtccaggtacccggcggccgtcgcgcgcctgccgcgcgtgtggcgtgcgccccgcgccgtgggggcgggaacccccgggcgcctgtggggtggtgtccgcgctcgcccccgcgtgggcggcgcgcgcctccccgtggtgtgaaaccttccgacccctctccggagtccggtcccgtttgctgtctcgtctggccggcctgaggcaaccccctctcctattgatcat

SEQ ID NO: 9452 - RNA, 341 nt, Homo sapiens
  source 1..341: mol_type = other RNA
aggctgggctgggacggagggcaacttcccctacactaccctttccacccagccccagggagccaggcacctccagcgggatttaataggagactgggcatggggacggccgggcacagtggctcacgcctgtaatctcgatactttgagaggtcgagtggggaggattgcttgaggccaggagttcaagacgagcctggcaacatggcgataccctggctctatttaagaaaccaataattaaaaaaaaaaataaaaataggatactgggcgtagagggcggggccaatgaggagtctttacgggtcgtcaaccctagaaagggggtgccctgggccttc

SEQ ID NO: 9453 - RNA, 1908 nt, Homo sapiens
  source 1..1908: mol_type = other RNA
agggaaggaggcttggtcttagtcctacgtaatccctccatgatgcatacctgaaagtatctcctcttccagtctcccatttcaacactgggatccatcccatccagggtcatttactggtactgcttctcttccagtcggataaagtttgccccctttcctgacactatatgtgaaacaaagctcatccccaaatctctctgctacttgcagagcagcctgcttctcagtgttcatcaggatctgattcaaaagtaacacaatgtctctccaagagagttcaaatacctgggttaaattctggaaagcctctatctatctgtcagggtcatgtgaaaacttgccaaaaatcccccttaatgtactttaagtcctgtagggggaaggagacctgcaccttactggggccaaattcacctggcatctgttggaagaggaggagtgagactggggcttgtctagggtgaggatttctaggattaggcaagcgagagactgaagctggatagagaggttgaggtggacccagaggagcagagctggagggagctggcttctctgctgggagtgcctctgggatttgtttctttagttccctggaattgccctttgcagcctctcctgaaatgacaaagcaggagggctggatcaatcctacactgtcagcaaagatctagatttccctgcaaggtataaaaagcctgcacatgtggggcctcaggccattcgtcctcacgcctacagaaaatgtccagctgccagatggtatcacaatgaatggttccttcctgagaccaagccagtccttcataatttggccaaacctttgttccgagggctaggaggtgtttttcctccagattctgagggtcaaagcagactcagtggttcaggatacacaggctaggaggtgtttttcctccagattctgagggtcaaagccatctcagtggttcaggatacactccagaggagaataagctgggggtggtgaagagagctggttgcccattttgtggtactggtttaataggtttttccatcaagcctccaatataaacagtgttgggaagcaggggccgggcaaaatcaaaggcaaaatcagagttaacaaaccacaactctgctttcagtagaagatgagacaaaactggcctagagccttctgggaaatgctccttgatggtgttgtcaaatgtagactgcatgtcccattggctcctggagaaactaaagaacatcagaaaattcttcactcggccccagaagtccatgtgatcagtcagcaaggaagggaatactggaacataagacaaggggcttggtagcccaaaatccaaagagccgaatgtggtgggaagaatggccacaaatggtttcacaagcttctcagcaatcaggaaagaacagaaatcaaatgcttcaacaaataccagatcatagttctcattctttaaggaatccattatatcctttctgcttagcaaataactacattgagtcccaaatatttccattagctttacaagggcttcagattcttttctgccatccaatgctgtttctatgtagctatcaaaatgcttcttaattcttttttgatgatcttcaggtgaaaaccacctgataacttggtatgatttttcctcctctttaatatctgggatcaaaaactttccactctgatgaagcatagtcacattatgaccatgctcttgaagaatctgagacacccggtccaacagtaggtaatggcttccacacagccagtatttctcagttgtgggtctctgcagtgccttctttagtattcctgtaggtccagacagccaatatttggatatttgcctttatggatatgtggactcatgcctctttccagtggctctggtctaccatggtgggtat

SEQ ID NO: 9454 - RNA, 3503 nt, Homo sapiens
  source 1..3503: mol_type = other RNA
agggaaggggacgagggttggggatccacttccaagctcactcccaaccacgtctctcaccacatgggactctttacaggactgcgttaccatgtggcagctgtcttccccttgtgcagctgtgctctttgaatgaatgaatcatgttagaatgaaattctggtgtatttatggagaactttttcctttgaagcctaaacacattttgattggtcgtatttaaattccaacaagccttttcctgccttcacactggcttcaggcaacagatccccatcaggcatgtctctcactgcacacagatgttcacacactgggaaagaatgtgactccaaggagagcagctcagaatcttcaggccagaacatgtgtaatttgccacaccaatgttctccattaaaaattactacctcagtccacccctctctttatcattttacacataaaacatggcagcagaggggtaagggattcacttaaggtcacataccaatatgtgtcacaacttgaactatgtgtgccggggtcttctgatcccccatgtccagtgctggttttgctacagctgaccagccccttgcacactcacagtagaactggaactagctcctcaaagagtgaggcagagctggagacgagtgccccagggtcccctgctgcagggaatcaaagaccccgtcacaattagcttagtaaaaccaacactatctggtgtcccatatccgcaagcacttaaaatgtcgttccaatcttcaaagaaattctttcattccatttttatctgcttttacccaggacattgtttcccagctccccagtagttcactaggtgatttgcatctcattagaagctccagaagtgacatctcccagactgctgcctggcattgtgggtccctaagcatcagatctaggtcttggattttccaagttgacacttttttaaaagctgagttaatgctgttttcccactgggtgcagtttgggtggccattttcgccataattcctgctcccgtgctggatcaaggttagggaactgccattgtcaaagatgaagtcagtcatctccacgtgaaagtacgtggtggatgagaatattctggggcctcagaataaaggagtttaaagactcctaaaaatagaaagatgctacatgatgcagatattctgaacactacacaaagcaaaacaaaaagacagcaagacaatagcaaaccattgctgaagctgtataattgattctaaacgtttgccttttaaacattttcccctggatccaatcctcctgagaccgcagagtttttgccctacatttatattttgctttaaagatagtctccctaggtcagaatgcctttttggctttgtcatttcttcatactacaacctccagaagagcactgaacagcactgtacctctggaaaccagagatagtatttccatggtcagcaaaattgttctcttggaataagagaaatgattttcccagtgtccagggaaataaggagcccttatgtctactttgggctcaagccatttgatgcagcttccagcacaaagcaagtgcctgatggtgcctagagcttccgccatccagaattccttttgtccagtgaatacttccctgagcttatgccaccttttcaaaatggcagatagctaatctgcagaattgatctaagctcttaggaaagggttaagtccatggtttttccaacactggctacaaattaaaatcactgggaaggaggaggaactttgttttaaacaagtaacaatgccagaaccctacccctgaccaattaaattaggatctccaggggtgaggtcatgatatctgtatttttaaaaagcccttcagatgattctaatatgcatccagggtggagaaccactccagtataacaagaaatacaacagccccttcgcagcacctgctaatgcctctggcaccatgttttatcttttcatatattatctgtcattctcactacaaccctacaaggaagggtcatcattcccaagtgaaggcctctaataagtgctgaggtggttatcatactccagtttttctgacttcagattcccaccccaacacacgtttctcaaagtgtgggacatgggccactagtggtcaccaagttgactcttgatgacgtatggatgtggcattaaataacataattcttttacataatttcttatgtaaaataaagttacttttttcaattctcaatttaaatcctccagattactttaaggagaaagtcttaatggtgctagtatgtcttaaattcctctcacatttactcatctctctttttaacaagccttttaagaaacccagaaccttctataggaaatggaatctagcacaagtgtgatgataccatttcactttcaccgtatttactatatagttcacttctatatatggcaaatgacactggttttccatttacagtggcgaataaagttccagttttaaagacatgtatttaagcaaaaaaaaaaatcagttgaattttaaaaatattaaatagtagtacaggtgaataaagtaaaaaatgcctaagaggtagatacgtgacaaaagtttgagaaatattcccctacaacatgctaatttttaaaacaggcatacccacacctgttagccaacgggactgctcatctaccatcctactccaatagactggcaacaacctgttccgtccactttacatccactcacgacctgtgaactttgctgctgtttccaactgaagaggaatcctttggccagtaattcttcttttagaaatttatcctgatgaaggaccacaggagggtgccagggtctatggctctcccaggatattctctccctttcttcccaggacccctgtgcgttgcctgcccattcctcaggagccaagaacgcattctgccccaccaagctggggaatacgtgggctgcatgctccatcctgcccttccttgcagttgtccttcacttccttcaagcttgctaggaaatttaccagaactggcacatcatggacggaattcctgccgtattagaaagtctgagggagagtggatgtcagacctccagagcatacttcacaccagcagccggacctaaggacacttctcttcattgatctggccacttgatctgagatgagccattcaattttatgggcctcagtttctcttcaaagacctcgcaatttgcagcagggatttgagcctgggcagtgactccagagtccttaattactattttatgctgccatgtagacaccttcagcctccataagaagcctacagaaggggcctggtggtggttccatgaagaaagttgtggagactccagattgtatgcttcaagcactgggtcagcagctgaaatatcacggtgaccaagacaaacaagatccctgctctcttggagcttacacggcctcacgtcttcatttatagaaagagaagcattagccaggcatggtggtgtg

SEQ ID NO: 9455 - RNA, 3212 nt, Homo sapiens
  source 1..3212: mol_type = other RNA
agggaaggggacgagggttggggatccacttccaagctcactcccaaccacgtctctcaccacatgggactctttacaggactgcgttaccatgtggcagctgtcttccccttgtgcagctgtgctctttgaatgaatgaatcatgttagaatgaaattctggtgtatttatggagaactttttcctttgaagcctaaacacattttgattggtcgtatttaaattccaacaagctgaaaagcaaaagcatttatgtcagtttcacagatgaggctccaagaggttaactggcgattactctggagttacagcatcttaaagttggaagggactttaaagggcctctgggctaatggttcttacccttttcctgccttcacactggcttcaggcaacagatccccatcaggcatgtctctcactgcacacagatgttcacacactgggaaagaatgtgactccaaggagagcagctcagaatcttcaggccagaacatgtgtaatttgccacaccaatgttctccattaaaaattactacctcagtccacccctctctttatcattttacacataaaacatggcagcagaggggtaagggattcacttaaggtcacataccaatatgtgtcacaacttgaactatgtgtgccggggtcttctgatcccccatgtccagtgctggttttgctacagctgaccagccccttgcacactcacagtagaactggaactagctcctcaaagagtgaggcagagctggagacgagtgccccagggtcccctgctgcagggaatcaaagaccccgtcacaattagcttagtaaaaccaacactatctggtgtcccatatccgcaagcacttaaaatgtcgttccaatcttcaaagaaattctttcattccatttttatctgcttttacccaggacattgtttcccagctccccagtagttcactaggtgatttgcatctcattagaagctccagaagtgacatctcccagactgctgcctggcattgtgggtccctaagcatcagatctaggtcttggattttccaagttgacacttttttaaaagctgagttaatgctgttttcccactgggtgcagtttgggtggccattttcgccataattcctgctcccgtgctggatcaaggttagggaactgccattgtcaaagatgaagtcagtcatctccacgtgaaagtacgtggtggatgagaatattctggggcctcagaataaaggagtttaaagactcctaaaaatagaaagatgctacatgatgcagatattctgaacactacacaaagcaaaacaaaaagacagcaagacaatagcaaaccattgctgaagctgtataattgattctaaacgtttgccttttaaacattttcccctggatccaatcctcctgagaccgcagagtttttgccctacatttatattttgctttaaagatagtctccctaggtcagaatgcctttttggctttgtcatttcttcatactacaacctccagaagagcactgaacagcactgtacctctggaaaccagagatagtatttccatggtcagcaaaattgttctcttggaataagagaaatgattttcccagtgtccagggaaataaggagcccttatgtctactttgggctcaagccatttgatgcagcttccagcacaaagcaagtgcctgatggtgcctagagcttccgccatccagaattccttttgtccagtgaatacttccctgagcttatgccaccttttcaaaatggcagatagctaatctgcagaattgatctaagctcttaggaaagggttaagtccatggtttttccaacactggctacaaattaaaatcactgggaaggaggaggaactttgttttaaacaagtaacaatgccagaaccctacccctgaccaattaaattaggatctccaggggtgaggtcatgatatctgtatttttaaaaagcccttcagatgattctaatatgcatccagggtggagaaccactccagtataacaagaaatacaacagccccttcgcagcacctgctaatgcctctggcaccatgttttatcttttcatatattatctgtcattctcactacaaccctacaaggaagggtcatcattcccaagtgaaggcctctaataagtgctgaggtggttatcatactccagtttttctgacttcagattcccaccccaacacacgtttctcaaagtgtgggacatgggccactagtggtcaccaagttgactcttgatgacgtatggatgtggcattaaataacataattcttttacataatttcttatgtaaaataaagttacttttttcaattctcaatttaaatcctccagattactttaaggagaaagtcttaatggtgctagtatgtcttaaattcctctcacatttactcatctctctttttaacaagccttttaagaaacccagaaccttctataggaaatggaatctagcacaagtgtgatgataccatttcactttcaccgtatttactatatagttcacttctatatatggcaaatgacactggttttccatttacagtggcgaataaagttccagttttaaagacatgtatttaagcaaaaaaaaaaatcagttgaattttaaaaatattaaatagtagtacaggtgaataaagtaaaaaatgcctaagaggtagatacgtgacaaaagtttgagaaatattcccctacaacatgctaatttttaaaacaggcatacccacacctgttagccaacgggactgctcatctaccatcctactccaatagactggcaacaacctgttccgtccactttacatccactcacgacctgtgaactttgctgctgtttccaactgaagaggaatcctttggccagtaattcttcttttagaaatttatcctgatgaaggaccacaggagggtgccagggtctatggctctcccaggatattctctccctttcttcccaggacccctgtgcgttgcctgcccattcctcaggagccaagaacgcattctgccccaccaagctggggaatacgtgggctgcatgctccatcctgcccttccttgcagttgtccttcacttccttcaagcttgctaggaaatttaccagaactggcacatcttgttggccacgctggttttgaactcctgacctcaggccat

SEQ ID NO: 9456 - RNA, 425 nt, Homo sapiens
  source 1..425: mol_type = other RNA
agggactgccttaggagaaagttctgaatttgttctcttcacagccagggcattgttgtaatcagacaccttctgttaaacgttactcaatttcaattctttgcttggccattctgagtcagagtgatcctcctgagtcactgttgcatcagacatggctcttgtgccactctctgctttgtgtatgttggtcttgtctgcccatttagacttcaagttcctctgtctctcctgctggtgtccacggtccatcaaggtctcaggtttgtccccactgtgctgttgctgctgatagtggcctcttgtcaggcatcttctgatccaggaccttgcccactttagcgaagatcagattctcatgagaatcaggggaaggaaggtagagtccaagttctggaggctggaagtccaagaccaaggcgttg

SEQ ID NO: 9457 - RNA, 78 nt, Homo sapiens
  source 1..78: mol_type = other RNA
agggactgccttaggagaaagtttctggaagttctgacattccagaaactttctcctaaggcagtccctgggagtcac

SEQ ID NO: 9458 - RNA, 78 nt, Homo sapiens
  source 1..78: mol_type = other RNA
agggactgccttaggagaaagtttctggaatgtcagaacttccagaaactttctcctaaggcagtccctggagtcacc

SEQ ID NO: 9459 - RNA, 408 nt, Homo sapiens
  source 1..408: mol_type = other RNA
agggagggtgtggtatggatgtagaccaaaacaatcactaagaggttaagtactgttccagctatacctaacatagtcaagatagattcttctttttcttctcttcttgcttcttaacatcttctgctgtagtgatgacagaagtaccagttttcccagaaaatgtcttcattgttcattaaatggaagtggatcatcataaaagtcttcatactcagagtcttcatgttgagtagcctaatgaggaagaagtgatgaggttggtcttgctgtctcaggctggcagaaaatctgtatataagtggactagtgcagttcaaacctgtgttgttcaagggtcagctgtaatttttttgagacggagtttcactcttgtggcccaggctggagtgcaatggcatgatcttg

SEQ ID NO: 9460 - RNA, 1105 nt, Homo sapiens
  source 1..1105: mol_type = other RNA
agggcatgtccagggggtccaggtctgctctgtagtagccattgcggcagacacagttggtggccccttcagaagtggtccggctgttgatgggacagtgggtacaggcctcatccccttggttggccttgaaagtcccagatggacaacctcggcagacggtgccattctcaacggcctcgaagcctgctttgcacatgcagcgcccgatgggcaccagccactcgccgtccccgttacagtagagcttgatgggtacatccacctcttccgcattggcgatgcagctgccccgggcagccaccagcgatgtgctctcagcccccgacagggtttcctggaagatggcgccattctggatgatgcgggggcacttgcggtagaagacacgcacggcgatgagggacatgcagccgccatagtcctggaaggccaggtagaagccgctgcgggacacaggtccgaagctccgcacctcggtgttgattttcatgacgcggccacccaggtccacctgggagaagctctcgtcggctgcaatggtatccaccttcacccatggattctccatccagttggggaaggtcttggtggccgagtcaaagtcagcctcatagtaatagaggttgaaggtctccttgcaggagccaggcacgctggggatgctgctgcagtcacgcaccgaaaacttcatctccacgtggatgcggtgggcgccacggcgccggataaacttggtccgtagccagttgttctggcttgactcaaacacgttgcacacctggtacgtgcggatcgtgttcatgttctcatcgtagccactcacctcttcccaccctgatggaggatgcaccatccagcccagctcagcagtcgctgtagtggagtccattagcgtttcttccacggcggcgagcagcggcagcagcagcagcgcggcccccagcctccgcagagccatggctgcgcttcccggggcctcgggccgcggcgccgcggggcccggacggcccgggcgggagcgcgcgccccgggctcggggggccagggggggcggcaaggcgcggcgcacacacagccgccgccaccgcgcagccagcagaat

SEQ ID NO: 9461 - RNA, 1106 nt, Homo sapiens
  source 1..1106: mol_type = other RNA
agggcatgtccagggggtccaggtctgctctgtagtagccattgcggcagacacagttggtggccccttcagaagtggtccggctgttgatgggacagtgggtacaggcctcatccccttggttggccttgaaagtcccagatggacaacctcggcagacggtgccattctcaacggcctcgaagcctgctttgcacatgcagcgcccgatgggcaccagccactcgccgtccccgttacagtagagcttgatgggtacatccacctcttccgcattggcgatgcagctgccccgggcagccaccagcgatgtgctctcagcccccgacagggtttcctggaagatggcgccattctggatgatgcgggggcacttgcggtagaagacacgcacggcgatgagggacatgcagccgccatagtcctggaaggccaggtagaagccgctgcgggacacaggtccgaagctccgcacctcggtgttgattttcatgacgcggccacccaggtccacctgggagaagctctcgtcggctgcaatggtatccaccttcacccatggattctccatccagttggggaaggtcttggtggccgagtcaaagtcagcctcatagtaatagaggttgaaggtctccttgcaggagccaggcacgctggggatgctgctgcagtcacgcaccgaaaacttcatctccacgtggatgcggtgggcgccacggcgccggataaacttggtccgtagccagttgttctggcttgactcaaacacgttgcacacctggtacgtgcggatcgtgttcatgttctcatcgtagccactcacctcttcccaccctgatggaggatgcaccatccagcccagctcagcagtcgctgtagtggagtccattagcgtttcttccacggcggcgagcagcggcagcagcagcagcgcggcccccagcctccgcagagccatggctgcgcttcccggggcctcgggccgcggcgccgcggggcccggacggcccgggcgggagcgcgcgccccgggctcggggggccagggggggcggcaaggcgcggcgcacacacagccgccgccaccgcgcagccagcagaatg

SEQ ID NO: 9462 - RNA, 1174 nt, Homo sapiens
  source 1..1174: mol_type = other RNA
agggcatgtccagggggtccaggtctgctctgtagtagccattgcggcagacacagttggtggccccttcagaagtggtccggctgttgatgggacagtgggtacaggcctcatccccttggttggccttgaaagtcccagatggacaacctcggcagacggtgccattctcaacggcctcgaagcctgctttgcacatgcagcgcccgatgggcaccagccactcgccgtccccgttacagtagagcttgatgggtacatccacctcttccgcattggcgatgcagctgccccgggcagccaccagcgatgtgctctcagcccccgacagggtttcctggaagatggcgccattctggatgatgcgggggcacttgcggtagaagacacgcacggcgatgagggacatgcagccgccatagtcctggaaggccaggtagaagccgctgcgggacacaggtccgaagctccgcacctcggtgttgattttcatgacgcggccacccaggtccacctgggagaagctctcgtcggctgcaatggtatccaccttcacccatggattctccatccagttggggaaggtcttggtggccgagtcaaagtcagcctcatagtaatagaggttgaaggtctccttgcaggagccaggcacgctggggatgctgctgcagtcacgcaccgaaaacttcatctccacgtggatgcggtgggcgccacggcgccggataaacttggtccgtagccagttgttctggcttgactcaaacacgttgcacacctggtacgtgcggatcgtgttcatgttctcatcgtagccactcacctcttcccaccctgatggaggatgcaccatccagcccagctcagcagtcgctgtagtggagtccattagcgtttcttccacggcggcgagcagcggcagcagcagcagcgcggcccccagcctccgcagagccatggctgcgcttcccggggcctcgggccgcggcgccgcggggcccggacggcccgggcgggagcgcgcgccccgggctcggggggccagggggggcggcaaggcgcggcgcacacacagccgccgccaccgcgcagccagcagaatgagccatccagcccgggcagaacggggacccgggctccgccagcgctgggcacggcccacctgagccgc

SEQ ID NO: 9463 - RNA, 1199 nt, Homo sapiens
  source 1..1199: mol_type = other RNA
agggcatgtccagggggtccaggtctgctctgtagtagccattgcggcagacacagttggtggccccttcagaagtggtccggctgttgatgggacagtgggtacaggcctcatccccttggttggccttgaaagtcccagatggacaacctcggcagacggtgccattctcaacggcctcgaagcctgctttgcacatgcagcgcccgatgggcaccagccactcgccgtccccgttacagtagagcttgatgggtacatccacctcttccgcattggcgatgcagctgccccgggcagccaccagcgatgtgctctcagcccccgacagggtttcctggaagatggcgccattctggatgatgcgggggcacttgcggtagaagacacgcacggcgatgagggacatgcagccgccatagtcctggaaggccaggtagaagccgctgcgggacacaggtccgaagctccgcacctcggtgttgattttcatgacgcggccacccaggtccacctgggagaagctctcgtcggctgcaatggtatccaccttcacccatggattctccatccagttggggaaggtcttggtggccgagtcaaagtcagcctcatagtaatagaggttgaaggtctccttgcaggagccaggcacgctggggatgctgctgcagtcacgcaccgaaaacttcatctccacgtggatgcggtgggcgccacggcgccggataaacttggtccgtagccagttgttctggcttgactcaaacacgttgcacacctggtacgtgcggatcgtgttcatgttctcatcgtagccactcacctcttcccaccctgatggaggatgcaccatccagcccagctcagcagtcgctgtagtggagtccattagcgtttcttccagccaccgtcttccgtgtctctcgtatccagccatccaaaatttcctcctgcttgcagaagtcactttacctccctgaacactggtgacttgacctttctagatttttctgcctggaacgcctggcccttcttgctttgttagcctggctaacttctcttccaaaactgagctcaaagcctccttcttccttcttcctggcagctgtcctgactcctcctgctctggctgggttaagtaacaaagtcatggtcattcaatgaacatctcctccacccgatgtgtgccaggccct

SEQ ID NO: 9464 - RNA, 1941 nt, Homo sapiens
  source 1..1941: mol_type = other RNA
agggccagaggagcctggagtggcagccagcctaagatgccatgctgagggcattcccatgcccagaatcacttggctgaaaaacggcgtggatgtctcaactcagatgtccaaacagctctcccttttaggtaagaactgcccttggtagacgtctatgcgatattcccattcaaatcaagctgagactccaggaatggaaacgagaggtataatttgtttataagtcagacaggttaggagtgaacagatggctcccaaatttccctgttatctgggctcacacagatcttttggggctttctgacagcaatgatgagaagctgtcactcaggtccagctcaccctcagtgcatttcagatgtgccagcccttcctgggcgtataatcagggctgctggctgcccaggggctgggcagccctaacactctcaatggccccataaaggaaagtgagtgggtctccagctgagcagtccaccctgagcactgtcctgtctgcagccaatgggagcgaactccacatcagcagtgttcggtatgaagacacaggggcatacacctgcattgccaaaaatgaagtgggtgtggatgaagatatctcctcgctcttcattgaagactcagctagaaagacccgtaagtcgacacgcgtttatgcttctcactgagctggctgggaggtgttgggtggcaagggagggcaccaattgaccagggccacagctgccaaccatgagcccgtgaagacaggggtaagcctcatatccctctttgcataaagctggaattggagggcacccagaggtgagcaggccttccctggcaacctagacaactctggaaacagacagggagattccctggacagcagacagagcccaggaacacaaggaaacccaaatagtcgagtcccagctctgctttttacttgctgtatgccctgaacctctgcccttcatccacgtgatgtcccacagtggcccagaacctgacctgtgcacacatgcacaccattgggagtgtggtagcctttacactaggggtccagcccatcggtgtgctaagcgtgctctcctcataaccactgctccccaggtaggcctgcaggtgtgatttcatagacatgggtgttaatcatggtcaaagactccaggctaagccattttcatcaaagtagataatcagaagtatttcacgtggtcatcttaggagaatcctagttgaaagtcacttctcctgctggttgtccaggaaatctgggagagatgttgcttactcttgatcatccatgaaatgtgagaaattccattagcttctgtggtcctagggcatgatttcaaagattcacttaagaatcaaagggtctggagacctgaaagcatttgttcatgtccagagcttcccccaagatactgttcctagggcaatgagtggtatagattctgtaagtgatggactaggtaccaggatcttcataaatggaatcactgcagtgacggtttaacactgctttcttctttttccttgactccatcacactcctgctttcctcattctctgctgctgcagttgcaaacatcctgtggcgagaggaaggtaccaagcttcattgttttgcgtcatgcctgtgatcacgtgtgtttggttctatgatgggccgtctttccatgatctgccaccagctttcccacacaaagcagcccagaatctaggccacagagtagtctagggaaggatgctgagggtccaagactttcaggaagaacgaaggaaccctggagctggttcctgagtgaaaaacttagcctctgtgttcagacttttgccatgttggtctaggtccctttaagtaacatgcaggaaaataaggaacattattgaccactaattttatgcctctgggccgggcacagtggctcacacctgtaatcccagcac

SEQ ID NO: 9465 - RNA, 3357 nt, Homo sapiens
  source 1..3357: mol_type = other RNA
agggccccccctcaatcctgtaagctgcctccacacctgagactctcccaccctgcaccaggcttgctgtttaaatggagccctggaggaggctgggaaaagtcgtgagcttcttcacccacgccatcctgggtcacctggatcagcagtttgtagctactttaggagaggcccatctggggggctgtctgcctccccaagatcttttttttttttttttttgagttggagtctcactctgtcacccaggctggagtgcagtggtgcggcctcggctccctgcaacctccacctcccgggttcatgccattctcctgcctcagcctccccagtagctgggattacaggcgcctgccaccacgcccggctattttttttcttttttaattttagtagaggtggggtttcaccgtgttagccaggatggtctgatccgcccgcctcggcctcccaaagtgctgggattacaggcgagccactgcacccggccacctccccaagatccttaactctcaccttgcccaccttcagtcccctcatggtgtctttatcttggagttcagtggccccaactccctgcaaatccaggatctgagccatgtctctggaagtccagctgcttgggaacagagccaaggtgttcagggagggaggagaagcagggaccacagatgagtccttgtacttccaggggatgtagaggtgaggctaggggtggccagagcccctcaggctgttcctgttctgaggatggtgccagagttttgtccgttgccacagccaggtgaggcatcctgggggaggagttcctgtgctttggactacagtcatccaagtctccatagcttggggtctgtgcaggaggcagaaagccctggggcagcctgggccctggactcgtcgtctccgaggctataggaaccaaggccaggtcattggaggcaggggcttccagaatgtagctggcgtggccctggggcatgggcttctggaggagctgcaagatgcggctgaggtctgaggacacgcgggactccagcctgttcatctgggcctggagctgctctagcctggagcccagcttcagaggccagcaatctgggtcttcctgagggctttgggggctgtgccttgggggcatttcctgcagtagctcaggccagaggccagatgcatctgagatgctcaggggaggggctgcatctgactggttgtcactgagaaagaaaccttggtggtcttggctgccaggagcctgtcggggggatgagtggagacccccggctgcgtcccgcaggttgaaggtgacctccagcttactccagaagctctccgcaaaggccgggtacatgtccagcacctccagcagatctgcccgctggatcttgtgcaggtcgcagtaggtcagagcccgcacgtctgcactggacttgcctggctgggcatggaggctgacgggttccccaaagatgtcattctttcctaggatggccacgaccacgtcgtcgcgcaggatctcgatggagcctcgggagatgaagtagagggtggagagcacgtcgccgaggtgcaccagcgtgtccccaggcggcgcgtgggtggtcttgaacttgacggctagcgcgcgcaggcagcccttgccggcgccgctgaaagctgggcagtgctgcagcagtgcgcggtgcaggtgcaggcagatgtcagcctgcaggcactcggggaagcccttcagcaccgcgttcatgtcaatgccattggtgtaggaccaggcgtgctggaaatactcctccaggcgctggcgcagtgggttggggatctggtggaagcggatgaactccttgacacgcagcatctgcgtgtggtagcgcgcggtgcccgagtacaggcgctggatgatcgcggacacgttcccgaagatgctggcgtacatcagggagccgatgagcatgacgcagatggagaagaccttctcggagttggtgttgggcgagacattgccgaagcccacgctggtgaggctgcagatgcaggccagccagtgcgctatgagcgcgaaggtgcacatgagcaagaagagcacagccgccccatactcagagtagcggtccagcttccgtgctacgcgcaccagccgcagcagccgcgctgtcttcaatagcccaatcagggttgtggtctcatcggagccagtgcggaagatcaggaggtcgaaagggatggcggccaccatgtcaatgaggaaccagcccttgaagtagtggacggcgatgcggcgggggtggctgaccacctcatcattggtgttgacataggtggtgcggaagttgatgacgatgtccacgacgaacatgatgtccacgatgagatccaccacagtgaggggactgcaggtatagctgcaggccccacgccgtgattcgtcctgatcgctgagcaggaaggcggctgagtagggcgtgaagacagccgtgtagatgaccagcagcaggatgagccagtcccacacggccttgaaggggctgtagtgcaggatggtccagcggtggatgcgcggcgcctgcagcttgtactccggcagcacatccgcgcccagggacaggacctgggtgaccttctcagtgacgttctgtgtccgctccaccaccttatggggcgcgatgatctcaatctccgtggtggagctggagcggtgcttctccaagttgaactccacgaagttgagcgtgaactgtgggatctggctgatggtcctgtacttgcccctgcctgtgcctggccctggtccgcctggcctgccatgagagccctcggagcccaggaagctctgggacaacaggcgctgggacaagctgcggctgctgcacttggccaggagctgggccaggtcctcgaagttgagaatgaacatgatgacagccccgtcctcgttcttcacgggcaccacatctaccaggcagcggaagctggaggcatccttgcggtagtagaggatgtccaccttgcactcctcagcccccagcagggcctgcgctaggcgggacacggcgctgcttggtgtgttggggcctgtgaggaagtcgcaggtgcagggttgctgcatcacctccactcgggagtagccgaagagttcgcagaagccgtcgttgcagtaaatgatggcgcagttctccatctgagcattggcaatcaggaacttccgactttggccctcgaacttgcggatgatggtgtccaggtaagtgttttggggagcgacgtggcccctgcggaccggcatctttcggccgcggcccctgcccggagccacaggcgccactggctcccggcgtctccgtctgtcctcgggctcagcagcgt

SEQ ID NO: 9466 - RNA, 3492 nt, Homo sapiens
  source 1..3492: mol_type = other RNA
agggccccccctcaatcctgtaagctgcctccacacctgagactctcccaccctgcaccaggcttgctgtttaaatggagccctggaggaggctgggaaaagtcgtgagcttcttcacccacgccatcctgggtcacctggatcagcagtttgtagctactttaggagaggcccatctggggggctgtctgcctccccaagatcttttttttttttttttttgagttggagtctcactctgtcacccaggctggagtgcagtggtgcggcctcggctccctgcaacctccacctcccgggttcatgccattctcctgcctcagcctccccagtagctgggattacaggcgcctgccaccacgcccggctattttttttcttttttaattttagtagaggtggggtttcaccgtgttagccaggatggtctgatccgcccgcctcggcctcccaaagtgctgggattacaggcgagccactgcacccggccacctccccaagatccttaactctcaccttgcccaccttcagtcccctcatggtgtctttatcttggagttcagtggccccaactccctgcaaatccaggatctgagccatgtctctggaagtccagctgcttgggaacagagccaaggtgttcagggagggaggagaagcagggaccacagatgagtccttgtacttccaggggatgtagaggtgaggctaggggtggccagagcccctcaggctgttcctgttctgaggatggtgccagagttttgtccgttgccacagccaggtgaggcatcctgggggaggagttcctgtgctttggactacagtcatccaagtctccatagcttggggtctgtgcaggaggcagaaagccctggggcagcctgggccctggactcgtcgtctccgaggctataggaaccaaggccaggtcattggaggcaggggcttccagaatgtagctggcgtggccctggggcatgggcttctggaggagctgcaagatgcggctgaggtctgaggacacgcgggactccagcctgttcatctgggcctggagctgctctagcctggagcccagcttcagaggccagcaatctgggtcttcctgagggctttgggggctgtgccttgggggcatttcctgcagtagctcaggccagaggccagatgcatctgagatgctcaggggaggggctgcatctgactggttgtcactgagaaagaaaccttggtggtcttggctgccaggagcctgtcggggggatgagtggagacccccggctgcgtcccgcaggttgaaggtgacctccagcttactccagaagctctccgcaaaggccgggtacatgtccagcacctccagcagatctgcccgctggatcttgtgcaggtcgcagtaggtcagagcccgcacgtctgcactggacttgcctggctgggcatggaggctgacgggttccccaaagatgtcattctttcctaggatggccacgaccacgtcgtcgcgcaggatctcgatggagcctcgggagatgaagtagagggtggagagcacgtcgccgaggtgcaccagcgtgtccccaggcggcgcgtgggtggtcttgaacttgacggctagcgcgcgcaggcagcccttgccggcgccgctgaaagctgggcagtgctgcagcagtgcgcggtgcaggtgcaggcagatgtcagcctgcaggcactcggggaagcccttcagcaccgcgttcatgtcaatgccattggtgtaggaccaggcgtgctggaaatactcctccaggcgctggcgcagtgggttggggatctggtggaagcggatgaactccttgacacgcagcatctgcgtgtggtagcgcgcggtgcccgagtacaggcgctggatgatcgcggacacgttcccgaagatgctggcgtacatcagggagccgatgagcatgacgcagatggagaagaccttctcggagttggtgttgggcgagacattgccgaagcccacgctggtgaggctgctgaaggtgaagtagagggctgtgacatacttgtcctgcaccgaggggcccgaggctgggtcgctgccgttgtagcgcttgccaagctgcacacccaggctgtccagccagccgatcttgtgttctaggtagggccgctccacattgccgatggcgtaccagatgcaggccagccagtgcgctatgagcgcgaaggtgcacatgagcaagaagagcacagccgccccatactcagagtagcggtccagcttccgtgctacgcgcaccagccgcagcagccgcgctgtcttcaatagcccaatcagggttgtggtctcatcggagccagtgcggaagatcaggaggtcgaaagggatggcggccaccatgtcaatgaggaaccagcccttgaagtagtggacggcgatgcggcgggggtggctgaccacctcatcattggtgttgacataggtggtgcggaagttgatgacgatgtccacgacgaacatgatgtccacgatgagatccaccacagtgaggggactgcaggtatagctgcaggccccacgccgtgattcgtcctgatcgctgagcaggaaggcggctgagtagggcgtgaagacagccgtgtagatgaccagcagcaggatgagccagtcccacacggccttgaaggggctgtagtgcaggatggtccagcggtggatgcgcggcgcctgcagcttgtactccggcagcacatccgcgcccagggacaggacctgggtgaccttctcagtgacgttctgtgtccgctccaccaccttatggggcgcgatgatctcaatctccgtggtggagctggagcggtgcttctccaagttgaactccacgaagttgagcgtgaactgtgggatctggctgatggtcctgtacttgcccctgcctgtgcctggccctggtccgcctggcctgccatgagagccctcggagcccaggaagctctgggacaacaggcgctgggacaagctgcggctgctgcacttggccaggagctgggccaggtcctcgaagttgagaatgaacatgatgacagccccgtcctcgttcttcacgggcaccacatctaccaggcagcggaagctggaggcatccttgcggtagtagaggatgtccaccttgcactcctcagcccccagcagggcctgcgctaggcgggacacggcgctgcttggtgtgttggggcctgtgaggaagtcgcaggtgcagggttgctgcatcacctccactcgggagtagccgaagagttcgcagaagccgtcgttgcagtaaatgatggcgcagttctccatctgagcattggcaatcaggaacttccgactttggccctcgaacttgcggatgatggtgtccaggtaagtgttttggggagcgacgtggcccctgcggaccggcatctttcggccgcggcccctgcccggagccacaggcgccactggctcccggcgtctcc

SEQ ID NO: 9467 - RNA, 3359 nt, Homo sapiens
  source 1..3359: mol_type = other RNA
agggccccccctcaatcctgtaagctgcctccacacctgagactctcccaccctgcaccaggcttgctgtttaaatggagccctggaggaggctgggaaaagtcgtgagcttcttcacccacgccatcctgggtcacctggatcagcagtttgtagctactttaggagaggcccatctggggggctgtctgcctccccaagatcttttttttttttttttttgagttggagtctcactctgtcacccaggctggagtgcagtggtgcggcctcggctccctgcaacctccacctcccgggttcatgccattctcctgcctcagcctccccagtagctgggattacaggcgcctgccaccacgcccggctattttttttcttttttaattttagtagaggtggggtttcaccgtgttagccaggatggtctgatccgcccgcctcggcctcccaaagtgctgggattacaggcgagccactgcacccggccacctccccaagatccttaactctcaccttgcccaccttcagtcccctcatggtgtctttatcttggagttcagtggccccaactccctgcaaatccaggatctgagccatgtctctggaagtccagctgcttgggaacagagccaaggtgttcagggagggaggagaagcagggaccacagatgagtccttgtacttccaggggatgtagaggtgaggctaggggtggccagagcccctcaggctgttcctgttctgaggatggtgccagagttttgtccgttgccacagccaggtgaggcatcctgggggaggagttcctgtgctttggactacagtcatccaagtctccatagcttggggtctgtgcaggaggcagaaagccctggggcagcctgggccctggactcgtcgtctccgaggctataggaaccaaggccaggtcattggaggcaggggcttccagaatgtagctggcgtggccctggggcatgggcttctggaggagctgcaagatgcggctgaggtctgaggacacgcgggactccagcctgttcatctgggcctggagctgctctagcctggagcccagcttcagaggccagcaatctgggtcttcctgagggctttgggggctgtgccttgggggcatttcctgcagtagctcaggccagaggccagatgcatctgagatgctcaggggaggggctgcatctgactggttgtcactgagaaagaaaccttggtggtcttggctgccaggagcctgtcggggggatgagtggagacccccggctgcgtcccgcaggttgaaggtgacctccagcttactccagaagctctccgcaaaggccgggtacatgtccagcacctccagcagatctgcccgctggatcttgtgcaggtcgcagtaggtcagagcccgcacgtctgcactggacttgcctggctgggcatggaggctgacgggttccccaaagatgtcattctttcctaggatggccacgaccacgtcgtcgcgcaggatctcgatggagcctcgggagatgaagtagagggtggagagcacgtcgccgaggtgcaccagcgtgtccccaggcggcgcgtgggtggtcttgaacttgacggctagcgcgcgcaggcagcccttgccggcgccgctgaaagctgggcagtgctgcagcagtgcgcggtgcaggtgcaggcagatgtcagcctgcaggcactcggggaagcccttcagcaccgcgttcatgtcaatgccattggtgtaggaccaggcgtgctggaaatactcctccaggcgctggcgcagtgggttggggatctggtggaagcggatgaactccttgacacgcagcatctgcgtgtggtagcgcgcggtgcccgagtacaggcgctggatgatcgcggacacgttcccgaagatgctggcgtacatcagggagccgatgagcatgacgcagatggagaagaccttctcggagttggtgttgggcgagacattgccgaagcccacgctggtgaggctgctgaaggtgaagtagagggctgtgacatacttgtcctgcaccgaggggcccgaggctgggtcgctgccgttgtagcgcttgccaagctgcacacccaggctgtccagccagccgatcttgtgttctaggtagggccgctccacattgccgatggcgtaccagatgcaggccagccagtgcgctatgagcgcgaaggtgcacatgagcaagaagagcacagccgccccatactcagagtagcggtccagcttccgtgctacgcgcaccagccgcagcagccgcgctgtcttcaatagcccaatcagggttgtggtctcatcggagccagtgcggaagatcaggaggtcgaaagggatggcggccaccatgtcaatgaggaaccagcccttgaagtagtggacggcgatgcggcgggggtggctgaccacctcatcattggtgttgacataggtggtgcggaagttgatgacgatgtccacgacgaacatgatgtccacgatgagatccaccacagtgaggggactgcaggtatagctgcaggccccacgccgtgattcgtcctgatcgctgagcaggaaggcggctgagtagggcgtgaagacagccgtgtagatgaccagcagcaggatgagccagtcccacacggccttgaaggggctgtagtgcaggatggtccagcggtggatgcgcggcgcctgcagcttgtactccggcagcacatccgcgcccagggacaggacctgggtgaccttctcagtgacgttctgtgtccgctccaccaccttatggggcgcgatgatctcaatctccgtggtggagctggagcggtgcttctccaagttgaactccacgaagttgagcgtgaactgtgggatctggctgatggtcctgtacttgcccctgcctgtgcctggccctggtccgcctggcctgccatgagagccctcggagcccaggaagctctgggacaacaggcgctgggacaagctgcggctgctgcacttggccaggagctgggccaggtcctcgaagttgagaatgaacatgatgacagccccgtcctcgttcttcacgggcaccacatctaccaggcagcggaagctggaggctccactcgggagtagccgaagagttcgcagaagccgtcgttgcagtaaatgatggcgcagttctccatctgagcattggcaatcaggaacttccgactttggccctcgaacttgcggatgatggtgtccaggtaagtgttttggggagcgacgtggcccctgcggaccggcatctttcggccgcggcccctgcccggagccacaggcgccactggctcccggcgtctcc

SEQ ID NO: 9468 - RNA, 3600 nt, Homo sapiens
  source 1..3600: mol_type = other RNA
agggccccccctcaatcctgtaagctgcctccacacctgagactctcccaccctgcaccaggcttgctgtttaaatggagccctggaggaggctgggaaaagtcgtgagcttcttcacccacgccatcctgggtcacctggatcagcagtttgtagctactttaggagaggcccatctggggggctgtctgcctccccaagatcttttttttttttttttttgagttggagtctcactctgtcacccaggctggagtgcagtggtgcggcctcggctccctgcaacctccacctcccgggttcatgccattctcctgcctcagcctccccagtagctgggattacaggcgcctgccaccacgcccggctattttttttcttttttaattttagtagaggtggggtttcaccgtgttagccaggatggtctgatccgcccgcctcggcctcccaaagtgctgggattacaggcgagccactgcacccggccacctccccaagatccttaactctcaccttgcccaccttcagtcccctcatggtgtctttatcttggagttcagtggccccaactccctgcaaatccaggatctgagccatgtctctggaagtccagctgcttgggaacagagccaaggtgttcagggagggaggagaagcagggaccacagatgagtccttgtacttccaggggatgtagaggtgaggctaggggtggccagagcccctcaggctgttcctgttctgaggatggtgccagagttttgtccgttgccacagccaggtgaggcatcctgggggaggagttcctgtgctttggactacagtcatccaagtctccatagcttggggtctgtgcaggaggcagaaagccctggggcagcctgggccctggactcgtcgtctccgaggctataggaaccaaggccaggtcattggaggcaggggcttccagaatgtagctggcgtggccctggggcatgggcttctggaggagctgcaagatgcggctgaggtctgaggacacgcgggactccagcctgttcatctgggcctggagctgctctagcctggagcccagcttcagaggccagcaatctgggtcttcctgagggctttgggggctgtgccttgggggcatttcctgcagtagctcaggccagaggccagatgcatctgagatgctcaggggaggggctgcatctgggtgccctggagcacaaggtcctgcccccatggagttctggctcccaggacccaggaggctgtagcccttagaggggaactggggccccagctcatggggagaccctgactggttgtcactgagaaagaaaccttggtggtcttggctgccaggagcctgtcggggggatgagtggagacccccggctgcgtcccgcaggttgaaggtgacctccagcttactccagaagctctccgcaaaggccgggtacatgtccagcacctccagcagatctgcccgctggatcttgtgcaggtcgcagtaggtcagagcccgcacgtctgcactggacttgcctggctgggcatggaggctgacgggttccccaaagatgtcattctttcctaggatggccacgaccacgtcgtcgcgcaggatctcgatggagcctcgggagatgaagtagagggtggagagcacgtcgccgaggtgcaccagcgtgtccccaggcggcgcgtgggtggtcttgaacttgacggctagcgcgcgcaggcagcccttgccggcgccgctgaaagctgggcagtgctgcagcagtgcgcggtgcaggtgcaggcagatgtcagcctgcaggcactcggggaagcccttcagcaccgcgttcatgtcaatgccattggtgtaggaccaggcgtgctggaaatactcctccaggcgctggcgcagtgggttggggatctggtggaagcggatgaactccttgacacgcagcatctgcgtgtggtagcgcgcggtgcccgagtacaggcgctggatgatcgcggacacgttcccgaagatgctggcgtacatcagggagccgatgagcatgacgcagatggagaagaccttctcggagttggtgttgggcgagacattgccgaagcccacgctggtgaggctgctgaaggtgaagtagagggctgtgacatacttgtcctgcaccgaggggcccgaggctgggtcgctgccgttgtagcgcttgccaagctgcacacccaggctgtccagccagccgatcttgtgttctaggtagggccgctccacattgccgatggcgtaccagatgcaggccagccagtgcgctatgagcgcgaaggtgcacatgagcaagaagagcacagccgccccatactcagagtagcggtccagcttccgtgctacgcgcaccagccgcagcagccgcgctgtcttcaatagcccaatcagggttgtggtctcatcggagccagtgcggaagatcaggaggtcgaaagggatggcggccaccatgtcaatgaggaaccagcccttgaagtagtggacggcgatgcggcgggggtggctgaccacctcatcattggtgttgacataggtggtgcggaagttgatgacgatgtccacgacgaacatgatgtccacgatgagatccaccacagtgaggggactgcaggtatagctgcaggccccacgccgtgattcgtcctgatcgctgagcaggaaggcggctgagtagggcgtgaagacagccgtgtagatgaccagcagcaggatgagccagtcccacacggccttgaaggggctgtagtgcaggatggtccagcggtggatgcgcggcgcctgcagcttgtactccggcagcacatccgcgcccagggacaggacctgggtgaccttctcagtgacgttctgtgtccgctccaccaccttatggggcgcgatgatctcaatctccgtggtggagctggagcggtgcttctccaagttgaactccacgaagttgagcgtgaactgtgggatctggctgatggtcctgtacttgcccctgcctgtgcctggccctggtccgcctggcctgccatgagagccctcggagcccaggaagctctgggacaacaggcgctgggacaagctgcggctgctgcacttggccaggagctgggccaggtcctcgaagttgagaatgaacatgatgacagccccgtcctcgttcttcacgggcaccacatctaccaggcagcggaagctggaggcatccttgcggtagtagaggatgtccaccttgcactcctcagcccccagcagggcctgcgctaggcgggacacggcgctgcttggtgtgttggggcctgtgaggaagtcgcaggtgcagggttgctgcatcacctccactcgggagtagccgaagagttcgcagaagccgtcgttgcagtaaatgatggcgcagttctccatctgagcattggcaatcaggaacttccgactttggccctcgaacttgcggatgatggtgtccaggtaagtgttttggggagcgacgtggcccctgcggaccggcatctttcggccgcggcccctgcccggagccacaggcgccactggctcccggcgtctcc

SEQ ID NO: 9469 - RNA, 3170 nt, Homo sapiens
  source 1..3170: mol_type = other RNA
agggccccccctcaatcctgttggcaacactttctatcatattgaatttagtccccttgccttgattttataaaaaaaaaaaaagtgccatacccttcatttttcagctttagtatggaagaatgccttaatattataaatatgacctgtaaatctaattattcgaagccaagtttattgctttagatctatcagaatggtactttttccaccattttggaaaaaatgacttaggcatgtgaaattcaagttgcaatacattatttttaaatcacaatttaccacaaagatagtgattctcaactttctcaaatgcctccaggattatctaaaaattccaaaaggttattattcgaaataatagcaagtgtaggaaaggtgtggttctttcagcagagagatgggtagcgaaataagatttccacagggctttataattccagggaggttggcagagaatctccttattctggggggtggtctttcctttgaggtcttggtttcctcactgccagtgtggaataggaaattgggctttgagaatgtcatagacttaattcaattcttttttttttttttggcctctgatttctggtttgtataagtgttgctgctgtcttctcacagaaatgatataagaaattatcaccaaagtaacactgtaatgttgaggctaagcttgtcaacctgatcgttatttttttctatagtctttgcacatctctatagtctttcatgaggacttcatgttcccctatattttaccttctctttttaataactgcagtgttacacttccagttttattactcatactttctaagagcagaacatgacatgtaaatatacgagtccttttcctattataggtctttgaatatgaatttactgctctcctgtttccacattcattttttcattttgatacttttcttataccaccaagacactatctcatcttgccctaataaaaatgaattgatttctttatatatttatccatttatttaacaagtacttattgactacttactatatgtcatacactctgctaggcactgagggtgcaatgatgtttaagatacatttccctaccctgaaggactcactcttgtaatggggaacacaaggtcagctggtggacaccagatggtacctgacaactcctttccttggacatttaagaaacattgttcagatacttattgcttatcccagaggaagcccatggcccttggcaaggttttgttgttgtttcacactctatggtcttatagtctcatggtcacctcattctacaattgattttacttgtttttcgccttccgtggctatcctattttctatgccatgcacagaccgtatgtggaattcagtccccttttcttgatttcctatgaaacataaggcattaatgcatgtagtgtgcattattaaaggtttcaggtgatgtgatgacaaaggacacatggaaaataattaaacttgagtgttactctctttttagaatttcttaggtcaattctactatcaggagctggccgattttgcgctaatgacctcccatatgtgggtgttgtctgatcctttgctccctctacagtgtccttgtatttggaatttgcttccaattcccttaattctttctcattttgaatgcaaggcaattttattctttgtttcactgaaccattccaaatcatactctggaggtctctccttttacagccacaatggactaggaaccaattttgttaagtagaaggctttctactctatgcaaaaaattttacacttccttaggggctgaagtggctgcagtcagtgttggttttaaatagtgatgtagttttcccctcccttacatatgtgaactatatatggtgctgggaatcactgtagagatcttagaccatgctatgtgctgtgggagtcagagaaggtacttcagaaagtcaggaaagcttcccagagatgagatctgaactggttttaaaatatgaggacgaatttacctttctgtcaactaaggctttgttgctgtcagactcctggagtttggttttctcttccttaaacctgagttctctcaggaagcatctgggtcattctgcaatggccagcaggctggctgccacagtaattagccaaacatgtccagacatgttgcatactcaagctgggagctcagcttctggtgatgaagtaatcaagtgtcataatagaaaagaagctgacgaattcagatcgctatcgtttggtggatggagcaaccaaggttgagagaggtaaaattatttggtcaagaacatacactggttagtgacagaactcacaaagccgtcatctcctgatatcttgacaagtgctctttccacttcagagttctgtctgtctttaccagatgaggatatacttcatattatatcatcttccttggtatcattcaagttagctcactcctggtctttctttatagtctcagtctcgtctcttcacattataatcatcatgtgtgatgtcagggcccatggcttttaataatgtaccaacctggctttagagttccctgacatccttaacttcactaattatcatccgatgacagcaatctatatccatgggcacacctattatcttattgttacatacaactgttccacttctggaattctaaattccattttagtctaacctctaaacctaatttatatttgcctttgacctcatggaaattcttgatccagtcatttcttcctagcttttacctccttaattactcaaattttcctcctatttagatctcttttgcctatttatatctagctgagattccatccactataagaaaaagaagattcaaccagtagtttagtttaaataaatagttgcttatttttctcatgtaatagaacatttagaggtaggagtttactttaagggtttttgatgctctggagtgttttgctagggctgtaacaaagtaccacagtctgagtgatataatcaacaggaatttattgttccagagttctagagactagatgtccaaaatgaagatgtcgatctgcatttcattgcttttcttcttatcttcatgataaatttcttagaagaatagcctttgtttgttgtcttcatctctttacctttcaatcactcttaatggt

SEQ ID NO: 9470 - RNA, 1169 nt, Homo sapiens
  source 1..1169: mol_type = other RNA
agggccgaagggtggaagctgccatgctggcctgtacatggtatttggacaaactcaagagggaccaagattctgttcctcagtattatttaatcagatgaaggaaagcaaggaatacagagacatgggctgtcactattactagatgctctctagaatgttctgagaaacaaagagaactggagaggagagtaagagatcatattaacatttctgcctcatattggaggcaagtagaggaaaagcaattgccaaaggcacagaaataaaaggaaatttgggtgggagtgctaaagaagctcaggctgtgtcagggaagacgctgcaggatgggtggcaggcaggaaaatgtaaaaccatgagaagacagtaggccctttctgggactctctgaactgttgacagagctgtcgtcctcattcatttgaatatattattcacctctatatcacagattctgtcctagaagctgagctaaaatggaatgaaacattaaaaatccaattggtaaaactgccacaagggagtctgctaaccacttggctggagatgaggcttggctgtgatagcttcaaaacttcggcaatccttcagcttctgtctagacagaaagaagtcccctttctccgcagttttgtttcctgtggtctcatttatccagtcaaccatagtccaaaaagaggtgaatacaatttactctttgtttatccagactataatttcttttctgtgacaagttttgcaaagtatgaccaagtatctttttgaaaatatagatgaaaagaattgaagcagtgtgtaaattctggccatcatgaattttctttgattttaagaaagttttttcccatctcaggctcaagctattactgtcttctgtatctagtccttcagaaggcatagaaataaaactatgatcacttgcgtccaggaggtcgaggctgcggtgagttgttattgtgccactgcactccagcctaggcaacagggagagaccctgtgagctcagcatctcaggccacttccacatcactgcacctccacatcaacacaagcctccataaagttttttggccggaagtccaaattcagggccagccatcgtggctcatgcttgtaatcccagcactttgggaggccaagggagaaggatcacttgaggctaggag

SEQ ID NO: 9471 - RNA, 535 nt, Homo sapiens
  source 1..535: mol_type = other RNA
agggcttagctgcttgtgagcaagttactaaattttctgagtctcagtttctgcttttgtaaaagtgagaaaggtaatatcgacctgataggttcgttgtgagtatgaaatgtattatgtacagagcttggttcatgttagatgttcccattttagtgagtttgtgtttatttggtttgggttttaggattgcttaatgcctcagttaagtggtcagatacagaaagggtgatttatatgaggctaatgaaacttaaactttagagccctttattttcacagacctcttccaaaggccctgaacctcattttgtattcgtaattttgtattcttttttggaaagacagaccactccaaattatgtgttttaggggcccacaaaacaaagatctgcttctggttaaataggatacatagctctcctaagtatcctctacatcaaaacttctttggtagtctctacacatacttctcttttttttgaggcagagtgttgctctgttgcccaggctggagtgcagtggcacagtctca

SEQ ID NO: 9472 - RNA, 536 nt, Homo sapiens
  source 1..536: mol_type = other RNA
agggcttagctgcttgtgagcaagttactaaattttctgagtctcagtttctgcttttgtaaaagtgagaaaggtaatatcgacctgataggttcgttgtgagtatgaaatgtattatgtacagagcttggttcatgttagatgttcccattttagtgagtttgtgtttatttggtttgggttttaggattgcttaatgcctcagttaagtggtcagatacagaaagggtgatttatatgaggctaatgaaacttaaactttagagccctttattttcacagacctcttccaaaggccctgaacctcattttgtattcgtaattttgtattcttttttggaaagacagaccactccaaattatgtgttttaggggcccacaaaacaaagatctgcttctggttaaataggatacatagctctcctaagtatcctctacatcaaaacttctttggtagtctctacacatacttctcttttttttgaggcagagtgttgctctgttgcccaggctggagtgcagtggcacagtctcag

SEQ ID NO: 9473 - RNA, 537 nt, Homo sapiens
  source 1..537: mol_type = other RNA
agggcttagctgcttgtgagcaagttactaaattttctgagtctcagtttctgcttttgtaaaagtgagaaaggtaatatcgacctgataggttcgttgtgagtatgaaatgtattatgtacagagcttggttcatgttagatgttcccattttagtgagtttgtgtttatttggtttgggttttaggattgcttaatgcctcagttaagtggtcagatacagaaagggtgatttatatgaggctaatgaaacttaaactttagagccctttattttcacagacctcttccaaaggccctgaacctcattttgtattcgtaattttgtattcttttttggaaagacagaccactccaaattatgtgttttaggggcccacaaaacaaagatctgcttctggttaaataggatacatagctctcctaagtatcctctacatcaaaacttctttggtagtctctacacatacttctcttttttttgaggcagagtgttgctctgttgcccaggctggagtgcagtggcacagtctcagc

SEQ ID NO: 9474 - RNA, 539 nt, Homo sapiens
  source 1..539: mol_type = other RNA
agggcttagctgcttgtgagcaagttactaaattttctgagtctcagtttctgcttttgtaaaagtgagaaaggtaatatcgacctgataggttcgttgtgagtatgaaatgtattatgtacagagcttggttcatgttagatgttcccattttagtgagtttgtgtttatttggtttgggttttaggattgcttaatgcctcagttaagtggtcagatacagaaagggtgatttatatgaggctaatgaaacttaaactttagagccctttattttcacagacctcttccaaaggccctgaacctcattttgtattcgtaattttgtattcttttttggaaagacagaccactccaaattatgtgttttaggggcccacaaaacaaagatctgcttctggttaaataggatacatagctctcctaagtatcctctacatcaaaacttctttggtagtctctacacatacttctcttttttttgaggcagagtgttgctctgttgcccaggctggagtgcagtggcacagtctcagctc

SEQ ID NO: 9475 - RNA, 541 nt, Homo sapiens
  source 1..541: mol_type = other RNA
agggcttagctgcttgtgagcaagttactaaattttctgagtctcagtttctgcttttgtaaaagtgagaaaggtaatatcgacctgataggttcgttgtgagtatgaaatgtattatgtacagagcttggttcatgttagatgttcccattttagtgagtttgtgtttatttggtttgggttttaggattgcttaatgcctcagttaagtggtcagatacagaaagggtgatttatatgaggctaatgaaacttaaactttagagccctttattttcacagacctcttccaaaggccctgaacctcattttgtattcgtaattttgtattcttttttggaaagacagaccactccaaattatgtgttttaggggcccacaaaacaaagatctgcttctggttaaataggatacatagctctcctaagtatcctctacatcaaaacttctttggtagtctctacacatacttctcttttttttgaggcagagtgttgctctgttgcccaggctggagtgcagtggcacagtctcagctcac

SEQ ID NO: 9476 - RNA, 71 nt, Homo sapiens
  source 1..71: mol_type = other RNA
agggggaaagttctatagtcctgagatctaattacaggactatagaactttccccctcatccctctaccct

SEQ ID NO: 9477 - RNA, 5104 nt, Homo sapiens
  source 1..5104: mol_type = other RNA
agggggcgggctccggcgggaaggccaagtgcgcgcagggcctgtagggcgcggggggcggcccgggcgggggcgggggcgggggcggcgtggacggcggggaggctcggccggacccgttgaacagcgccaggccgggggacgcgggcctgtcgccgtcgcccttctggctcttggagtactgcggggacagcgggctcgacccctccggctgcacggggtacttgaggttggtctccaggactggcagcttcttcacctccaggggtgtcaggggcgactcgtcggaggcgggggagcaggtgacgggggtcggggggaacaccagcaggggcggccggtgcggcagcaggttggggaagggcggcgggatgtcgcacgcgtcccctgggggccccgccgcctcgtcctccggcgcgcggtggagcaggggcggcgatgcgccgtggagcaggaaggagcccgcgcccgggccgccgtcgtcgggcaggcaacacttcatctcctcgtacacggactccccggggtccgggctatcgggcctggccgcgtgccccagcatctcgatgtacacaggctcgctgtcgtcctcgtcacccggaggcgccgccgggggcagcgcgcactgcggagtcccgggggtcagaacgcgcgctgctgcccccggggcgcccgcgggcctcgcgtccccgggccgggaccccgatatctcctcgtaggagccgctgagcttggtgttggggctgcgcttgggctttcgaggaggaatcttcttcatggtgctgtagtcgtcgctgtgcggtctgggccgggccagagcttcgttggccgcttccctggccgcggagaggcaggcgctcacagcctcataggaagcactcagccgggtgttggggtccctctttggcttgggcgggggctgtttccgtggagacgggaggctgctgctgtcatccatgctgaacaccgagtgcagcgaaggagaccagatggacgggccaacgaggcactggcccaggccatccacggccgcgcagactgacatggagctggggtggaaatgcctgggtccactcttgtcatcggttcttttgcttccttcctcttgcatgttcctgacctctaacttctctttatggtagggagcgttcatttcactacggagccggtcattttcccgggcaatgtctgaagcattctgaatgaccagggcatcgtaggttttcagccccatgtcctctgtgttctgcagaaagctattgatagaagtcacctcttgttgtctgatgcttattctctgaagcaggtgctggcgtgctaaaaatcctctgataactttttggcaggttataatttttctctgcaactgtaggcacaaatcattgagttggtcagcatgccagtattttagaaacacttttcggactcccatctgccagccttgtaatttacactgctggagaacaagtcgacatcgctcggcagctgactgttccttcttctcacgcaggaatgtatcagccagtggcttataccttgacaggaaatccgagaaggaaaggcgaacagggtatccatatcggaagatcttcaccatctccaggaccccaatatattgtagctgagcagacacgtaaaaattatcaaaagtatctggcagctttgagttattgggcctgatgcaatgaatgaagtgtggagtgcacttctgaagttttccaataatatccattagtgatttcctgagttgtgatgctatggtgactggatctcctcgttccaatctttgaagaaatgtagaagttcctttcttttttaataacttactaagttctagataattcttgttttctccaataattgaagaagctgtcattttcttactgagcagggcagacttatgtcctcggaatttaaaggaaggataggcagatacgagggatcctgtttgtgacaatttcgactggaacaaatgattgatcacgacattttcactagttttcattacaaatagaagattctgtgaaagggagtctttatttttttcaatcgccccaacaacatcatacattacccttcctgcgtagtgcatgatggtgaaggctgtaccgtggtctttgagggcaacattcccattcccatccttcatgggggagtacaccgcatttgtgtttgaggattctaggagactttgtagtttttttggaaaatttgattccactgaccaaatcatttgactttcttcatccaataaggtgagaaatccagatggcttctggaaaaaaaagtccaaaactccattctggttaccaggagaatatgctgtttccatggtaactccctcttgtacacattccacttgctcgtggagaaaaagcacttcattgatatagtggtgcatcttctcattggtcatgttgacacaaagttgttcaaattcattcttttgaaactcttcaaaaccaaaaatgtccaatattccaatatccaatgtctgcatgcttttctgttcatcttgactgtggaggcaagaattcatggtattcaccaaaaagctaaacaaacgactgtacagggacttggccaagaggtctcggaaaaactcagcaatctgtatggtatgtcgtcgtattatcatatcccctttaaaatattgaatatcagttgttaaggcagatgccaattcatctgttgatacttgtaacattccagccacttgttccaggagctggaggtcagaaacgaaggcggagttcccctcattcagggcagtaaaccgaatgtctccaaggtgcaatattgctgctagaattacgaacagattctccacctccaagctgctgaagccaactacattcagggctcgtttcaaaacagccaatttctccctgttcagagaacgctcccctgtggatgcatcatcctgtatggtctggttcaaataccggtgtgcacataaattattaagatgaagtccatatttttcttcagcagataacccatccatcaacaagtagaaaatgagaaaattgctctggccaagaggttgtgaaacaagtctggatttctctagcaaatatgtataaattctggctccggttagctgttgtttcctctcacagaactgcagttcaaaatacttgatgaagcaactggacaaatcattaagtgtggtcttggcatgtccaaaggcttctaagatgcacacgacatgtttgaatctggaatccagtgtggccctgctggcgccagccctgcaggtgaggtgtcttatgatttgtttgctggcttcagactttcctgatcccctttctccactgaggatgaaacactgaggccgctgttcccggaagagctggtgaaaggctctctccacacaggagaagaggtgaggaggcagcgaggaacacagcttccctgaggagctgaaatacagctgggacaccatggaagaataaattggaagctccttgtatgggttaacaagcaaaagaatgtctccaatgaatgtatagatctgattgttcccaaagcgcttctgaatctcatagagcaggctgccatcattgagctcgctgagcgttgccaggtcatcgtttggggcaggaggcattagcttgacctgctcgggtttggtggaaccgctcatcatggggttttcagggatgctgtcctgagactgctgcttacacagaccttttgttgcatctttgaacataatgtctttttccaacaaactgtcttgcttggcaattggtaacaccaggggactgagcttactcgacagtacgggaagatcgtgaatgatctcttcatagggctcttcttgagctaaggtagaagcagataaaggctctttcattttttcttcccaggcaatttcggctttcagcagcatttcctcaataaactcagaggcagcaatatctgacgccttctcctcattacagttcacgaggtgtgggtttgcctgatgcatcaggagaagtttcaccagatttgtctggccatatttggctgccaagtggaggggagtccagtactgatcatctactatgttgaggtctccaccatgttccaggataagagacaccacctccttgtagccactcgcacacgccatgtgtaacagggttactccttcatcgtttttctcattgacatttcctccagatgataagaagtgtttgacatctgttaacatactcattggtctctgaagcttcatctggcgcagtgaggtcaaatccactccattttcatccagataggtcaacaggatagagctggattctgtcccttctacagcataatctaatgggatatttccattcacatcctggagaaggacattggctccagctaatacaagaagcaggacaatatcagggttatcgcaggcacaggcaatgtgcatgggcgtccagaagtcttcatcctggtggttgacgttgactcctctgtcaatcagaatttctgcaatgaaggcattatcataccgagcacacagatggagcagggaccctcccgaggagacgagggtgtgggggtctgccccctccttcaggagccgaagcacttctttgtcattgtggtggataatcgcgtcctgtagcatgtccgtgaggttgaagtgaactttcggattcttcgcatgcttcagccttttcaggaacccttcctgcttctgaaaagccttctcgcgctcatagtaggctttgatttgctcacagcgcatgcgcttcactagacgctgccgttggccaaggggaagggactctagcaagcactggtcgatttccatctcatgggatcgaaaaacgttacatagctgaaagcaacagcacttgataaaatgatagtgagacatctttccatctcagacaggaatcttgctacgggttccagcattctcttctgtcacaactgtcgttcccaggaaatgcattacttaaagcccttactcaggtaacagtttacctcaggatgcactattgcatggaggctctgttccatgatcctgcaaaaagcttcaaactcattctcattcggcagctggagttaagataagcctctccccggtgggtcttgaggcaccactggt

SEQ ID NO: 9478 - RNA, 5177 nt, Homo sapiens
  source 1..5177: mol_type = other RNA
agggggcgggctccggcgggaaggccaagtgcgcgcagggcctgtagggcgcggggggcggcccgggcgggggcgggggcgggggcggcgtggacggcggggaggctcggccggacccgttgaacagcgccaggccgggggacgcgggcctgtcgccgtcgcccttctggctcttggagtactgcggggacagcgggctcgacccctccggctgcacggggtacttgaggttggtctccaggactggcagcttcttcacctccaggggtgtcaggggcgactcgtcggaggcgggggagcaggtgacgggggtcggggggaacaccagcaggggcggccggtgcggcagcaggttggggaagggcggcgggatgtcgcacgcgtcccctgggggccccgccgcctcgtcctccggcgcgcggtggagcaggggcggcgatgcgccgtggagcaggaaggagcccgcgcccgggccgccgtcgtcgggcaggcaacacttcatctcctcgtacacggactccccggggtccgggctatcgggcctggccgcgtgccccagcatctcgatgtacacaggctcgctgtcgtcctcgtcacccggaggcgccgccgggggcagcgcgcactgcggagtcccgggggtcagaacgcgcgctgctgcccccggggcgcccgcgggcctcgcgtccccgggccgggaccccgatatctcctcgtaggagccgctgagcttggtgttggggctgcgcttgggctttcgaggaggaatcttcttcatggtgctgtagtcgtcgctgtgcggtctgggccgggccagagcttcgttggccgcttccctggccgcggagaggcaggcgctcacagcctcataggaagcactcagccgggtgttggggtccctctttggcttgggcgggggctgtttccgtggagacgggaggctgctgctgtcatccatgctgaacaccgagtgcagcgaaggagaccagatggacgggccaacgaggcactggcccaggccatccacggccgcgcagactgacatggagctggggtggaaatgcctgggtccactcttgtcatcggttcttttgcttccttcctcttgcatgttcctgacctctaacttctctttatggtagggagcgttcatttcactacggagccggtcattttcccgggcaatgtctgaagcattctgaatgaccagggcatcgtaggttttcagccccatgtcctctgtgttctgcagaaagctattgatagaagtcacctcttgttgtctgatgcttattctctgaagcaggtgctggcgtgctaaaaatcctctgataactttttggcaggttataatttttctctgcaactgtaggcacaaatcattgagttggtcagcatgccagtattttagaaacacttttcggactcccatctgccagccttgtaatttacactgctggagaacaagtcgacatcgctcggcagctgactgttccttcttctcacgcaggaatgtatcagccagtggcttataccttgacaggaaatccgagaaggaaaggcgaacagggtatccatatcggaagatcttcaccatctccaggaccccaatatattgtagctgagcagacacgtaaaaattatcaaaagtatctggcagctttgagttattgggcctgatgcaatgaatgaagtgtggagtgcacttctgaagttttccaataatatccattagtgatttcctgagttgtgatgctatggtgactggatctcctcgttccaatctttgaagaaatgtagaagttcctttcttttttaataacttactaagttctagataattcttgttttctccaataattgaagaagctgtcattttcttactgagcagggcagacttatgtcctcggaatttaaaggaaggataggcagatacgagggatcctgtttgtgacaatttcgactggaacaaatgattgatcacgacattttcactagttttcattacaaatagaagattctgtgaaagggagtctttatttttttcaatcgccccaacaacatcatacattacccttcctgcgtagtgcatgatggtgaaggctgtaccgtggtctttgagggcaacattcccattcccatccttcatgggggagtacaccgcatttgtgtttgaggattctaggagactttgtagtttttttggaaaatttgattccactgaccaaatcatttgactttcttcatccaataaggtgagaaatccagatggcttctggaaaaaaaagtccaaaactccattctggttaccaggagaatatgctgtttccatggtaactccctcttgtacacattccacttgctcgtggagaaaaagcacttcattgatatagtggtgcatcttctcattggtcatgttgacacaaagttgttcaaattcattcttttgaaactcttcaaaaccaaaaatgtccaatattccaatatccaatgtctgcatgcttttctgttcatcttgactgtggaggcaagaattcatggtattcaccaaaaagctaaacaaacgactgtacagggacttggccaagaggtctcggaaaaactcagcaatctgtatggtatgtcgtcgtattatcatatcccctttaaaatattgaatatcagttgttaaggcagatgccaattcatctgttgatacttgtaacattccagccacttgttccaggagctggaggtcagaaacgaaggcggagttcccctcattcagggcagtaaaccgaatgtctccaaggtgcaatattgctgctagaattacgaacagattctccacctccaagctgctgaagccaactacattcagggctcgtttcaaaacagccaatttctccctgttcagagaacgctcccctgtggatgcatcatcctgtatggtctggttcaaataccggtgtgcacataaattattaagatgaagtccatatttttcttcagcagataacccatccatcaacaagtagaaaatgagaaaattgctctggccaagaggttgtgaaacaagtctggatttctctagcaaatatgtataaattctggctccggttagctgttgtttcctctcacagaactgcagttcaaaatacttgatgaagcaactggacaaatcattaagtgtggtcttggcatgtccaaaggcttctaagatgcacacgacatgtttgaatctggaatccagtgtggccctgctggcgccagccctgcaggtgaggtgtcttatgatttgtttgctggcttcagactttcctgatcccctttctccactgaggatgaaacactgaggccgctgttcccggaagagctggtgaaaggctctctccacacaggagaagaggtgaggaggcagcgaggaacacagcttccctgaggagctgaaatacagctgggacaccatggaagaataaattggaagctccttgtatgggttaacaagcaaaagaatgtctccaatgaatgtatagatctgattgttcccaaagcgcttctgaatctcatagagcaggctgccatcattgagctcgctgagcgttgccaggtcatcgtttggggcaggaggcattagcttgacctgctcgggtttggtggaaccgctcatcatggggttttcagggatgctgtcctgagactgctgcttacacagaccttttgttgcatctttgaacataatgtctttttccaacaaactgtcttgcttggcaattggtaacaccaggggactgagcttactcgacagtacgggaagatcgtgaatgatctcttcatagggctcttcttgagctaaggtagaagcagataaaggctctttcattttttcttcccaggcaatttcggctttcagcagcatttcctcaataaactcagaggcagcaatatctgacgccttctcctcattacagttcacgaggtgtgggtttgcctgatgcatcaggagaagtttcaccagatttgtctggccatatttggctgccaagtggaggggagtccagtactgatcatctactatgttgaggtctccaccatgttccaggataagagacaccacctccttgtagccactcgcacacgccatgtgtaacagggttactccttcatcgtttttctcattgacatttcctccagatgataagaagtgtttgacatctgttaacatactcattggtctctgaagcttcatctggcgcagtgaggtcaaatccactccattttcatccagataggtcaacaggatagagctggattctgtcccttctacagcataatctaatgggatatttccattcacatcctggagaaggacattggctccagctaatacaagaagcaggacaatatcagggttatcgcaggcacaggcaatgtgcatgggcgtccagaagtcttcatcctggtggttgacgttgactcctctgtcaatcagaatttctgcaatgaaggcattatcataccgagcacacagatggagcagggaccctcccgaggagacgagggtgtgggggtctgccccctccttcaggagccgaagcacttctttgtcattgtggtggataatcgcgtcctgtagcatgtccgtgaggttgaagtgaactttcggattcttcgcatgcttcagccttttcaggaacccttcctgcttctgaaaagccttctcgcgctcatagtaggctttgatttgctcacagcgcatgcgcttcactagacgctgccgttggccaaggggaagggactctagcaagcactggtcgatttccatctcatgggatcgaaaaacgttacatagctgaaagcaaccacaatgtggatgagaggctccaaccagaaggaaaatacaacctttggaaatctctcctctgctttcactgaaagtctccgagcgcagttctggtccacgctcagagtctgacacatccctcccccgtccccacctctcaacacacacagctgatgaggccgattcctgtagatcgacttcaaaaaagaaaaagtcattccagaaaacacatcagctcaggctgactcaaaggcagccccaaattcagcccacagcggttggctgctgtccttttatgactggagagctggagtgcagctctttaattaaaagggaagccttagcctgctcaagg

SEQ ID NO: 9479 - RNA, 5038 nt, Homo sapiens
  source 1..5038: mol_type = other RNA
agggggcgggctccggcgggaaggccaagtgcgcgcagggcctgtagggcgcggggggcggcccgggcgggggcgggggcgggggcggcgtggacggcggggaggctcggccggacccgttgaacagcgccaggccgggggacgcgggcctgtcgccgtcgcccttctggctcttggagtactgcggggacagcgggctcgacccctccggctgcacggggtacttgaggttggtctccaggactggcagcttcttcacctccaggggtgtcaggggcgactcgtcggaggcgggggagcaggtgacgggggtcggggggaacaccagcaggggcggccggtgcggcagcaggttggggaagggcggcgggatgtcgcacgcgtcccctgggggccccgccgcctcgtcctccggcgcgcggtggagcaggggcggcgatgcgccgtggagcaggaaggagcccgcgcccgggccgccgtcgtcgggcaggcaacacttcatctcctcgtacacggactccccggggtccgggctatcgggcctggccgcgtgccccagcatctcgatgtacacaggctcgctgtcgtcctcgtcacccggaggcgccgccgggggcagcgcgcactgcggagtcccgggggtcagaacgcgcgctgctgcccccggggcgcccgcgggcctcgcgtccccgggccgggaccccgatatctcctcgtaggagccgctgagcttggtgttggggctgcgcttgggctttcgaggaggaatcttcttcatggtgctgtagtcgtcgctgtgcggtctgggccgggccagagcttcgttggccgcttccctggccgcggagaggcaggcgctcacagcctcataggaagcactcagccgggtgttggggtccctctttggcttgggcgggggctgtttccgtggagacgggaggctgctgctgtcatccatgctgaacaccgagtgcagcgaaggagaccagatggacgggccaacgaggcactggcccaggccatccacggccgcgcagactgacatggagctggggtggaaatgcctgggtccactcttgtcatcggttcttttgcttccttcctcttgcatgttcctgacctctaacttctctttatggtagggagcgttcatttcactacggagccggtcattttcccgggcaatgtctgaagcattctgaatgaccagggcatcgtaggttttcagccccatgtcctctgtgttctgcagaaagctattgatagaagtcacctcttgttgtctgatgcttattctctgaagcaggtgctggcgtgctaaaaatcctctgataactttttggcaggttataatttttctctgcaactgtaggcacaaatcattgagttggtcagcatgccagtattttagaaacacttttcggactcccatctgccagccttgtaatttacactgctggagaacaagtcgacatcgctcggcagctgactgttccttcttctcacgcaggaatgtatcagccagtggcttataccttgacaggaaatccgagaaggaaaggcgaacagggtatccatatcggaagatcttcaccatctccaggaccccaatatattgtagctgagcagacacgtaaaaattatcaaaagtatctggcagctttgagttattgggcctgatgcaatgaatgaagtgtggagtgcacttctgaagttttccaataatatccattagtgatttcctgagttgtgatgctatggtgactggatctcctcgttccaatctttgaagaaatgtagaagttcctttcttttttaataacttactaagttctagataattcttgttttctccaataattgaagaagctgtcattttcttactgagcagggcagacttatgtcctcggaatttaaaggaaggataggcagatacgagggatcctgtttgtgacaatttcgactggaacaaatgattgatcacgacattttcactagttttcattacaaatagaagattctgtgaaagggagtctttatttttttcaatcgccccaacaacatcatacattacccttcctgcgtagtgcatgatggtgaaggctgtaccgtggtctttgagggcaacattcccattcccatccttcatgggggagtacaccgcatttgtgtttgaggattctaggagactttgtagtttttttggaaaatttgattccactgaccaaatcatttgactttcttcatccaataaggtgagaaatccagatggcttctggaaaaaaaagtccaaaactccattctggttaccaggagaatatgctgtttccatggtaactccctcttgtacacattccacttgctcgtggagaaaaagcacttcattgatatagtggtgcatcttctcattggtcatgttgacacaaagttgttcaaattcattcttttgaaactcttcaaaaccaaaaatgtccaatattccaatatccaatgtctgcatgcttttctgttcatcttgactgtggaggcaagaattcatggtattcaccaaaaagctaaacaaacgactgtacagggacttggccaagaggtctcggaaaaactcagcaatctgtatggtatgtcgtcgtattatcatatcccctttaaaatattgaatatcagttgttaaggcagatgccaattcatctgttgatacttgtaacattccagccacttgttccaggagctggaggtcagaaacgaaggcggagttcccctcattcagggcagtaaaccgaatgtctccaaggtgcaatattgctgctagaattacgaacagattctccacctccaagctgctgaagccaactacattcagggctcgtttcaaaacagccaatttctccctgttcagagaacgctcccctgtggatgcatcatcctgtatggtctggttcaaataccggtgtgcacataaattattaagatgaagtccatatttttcttcagcagataacccatccatcaacaagtagaaaatgagaaaattgctctggccaagaggttgtgaaacaagtctggatttctctagcaaatatgtataaattctggctccggttagctgttgtttcctctcacagaactgcagttcaaaatacttgatgaagcaactggacaaatcattaagtgtggtcttggcatgtccaaaggcttctaagatgcacacgacatgtttgaatctggaatccagtgtggccctgctggcgccagccctgcaggtgaggtgtcttatgatttgtttgctggcttcagactttcctgatcccctttctccactgaggatgaaacactgaggccgctgttcccggaagagctggtgaaaggctctctccacacaggagaagaggtgaggaggcagcgaggaacacagcttccctgaggagctgaaatacagctgggacaccatggaagaataaattggaagctccttgtatgggttaacaagcaaaagaatgtctccaatgaatgtatagatctgattgttcccaaagcgcttctgaatctcatagagcaggctgccatcattgagctcgctgagcgttgccaggtcatcgtttggggcaggaggcattagcttgacctgctcgggtttggtggaaccgctcatcatggggttttcagggatgctgtcctgagactgctgcttacacagaccttttgttgcatctttgaacataatgtctttttccaacaaactgtcttgcttggcaattggtaacaccaggggactgagcttactcgacagtacgggaagatcgtgaatgatctcttcatagggctcttcttgagctaaggtagaagcagataaaggctctttcattttttcttcccaggcaatttcggctttcagcagcatttcctcaataaactcagaggcagcaatatctgacgccttctcctcattacagttcacgaggtgtgggtttgcctgatgcatcaggagaagtttcaccagatttgtctggccatatttggctgccaagtggaggggagtccagtactgatcatctactatgttgaggtctccaccatgttccaggataagagacaccacctccttgtagccactcgcacacgccatgtgtaacagggttactccttcatcgtttttctcattgacatttcctccagatgataagaagtgtttgacatctgttaacatactcattggtctctgaagcttcatctggcgcagtgaggtcaaatccactccattttcatccagataggtcaacaggatagagctggattctgtcccttctacagcataatctaatgggatatttccattcacatcctggagaaggacattggctccagctaatacaagaagcaggacaatatcagggttatcgcaggcacaggcaatgtgcatgggcgtccagaagtcttcatcctggtggttgacgttgactcctctgtcaatcagaatttctgcaatgaaggcattatcataccgagcacacagatggagcagggaccctcccgaggagacgagggtgtgggggtctgccccctccttcaggagccgaagcacttctttgtcattgtggtggataatcgcgtcctgtagcatgtccgtgaggttgaagtgaactttcggattcttcgcatgcttcagccttttcaggaacccttcctgcttctgaaaagccttctcgcgctcatagtaggctttgatttgctcacagcgcatgcgcttcactagacgctgccgttggccaaggggaagggactctagcaagcactggtcgatttccatctcatgggatcgaaaaacgttacatagctgaaagcaacctgccggagaagggtccgccggagccgggcgccaggcgacgcggcgatggccgggactcggctcggaaaccagccccgcgcggcgggtgagaggggtcggcagttgcccctgtgcccggggccggcgcggttgcgcgcagccaggccggctggaggctggggactgctccgccacccgctcggcggcggctctctc

SEQ ID NO: 9480 - RNA, 709 nt, Homo sapiens
  source 1..709: mol_type = other RNA
agggggcgggctccggcgggaccccagcgctgcaggcggtgcggctgagccagggagccccccgcgccctgcggctggatggtgaactcctcgccgtccagcaggaaggagccgctcagcccgcggcacaggctgaccgccgccagcgactcgggctccccattcacggtgccggagaagaagcagccgcgcagcccccgctcgcccccggtcgcccggccggagcccccgaggcgctcgatcttgaactcgggcgctaggaagctgtcgtcgggcgccaggcgcagcacgaagcccttgccgaaggcggacaggtggagcgcgagctcgcccgcgctgccgggcaaccgcgtgggcaccaccagctccgaggcctgccccccggctgcgggccgggccggggcgccgcgggccagcggcagcagcagcagcagcagcagcaggagcggaggccaccggggggcggcgggggcggggagcatgggggctgcggcggtggctgcgcgcaggagagggaagaagcccgccaggcgcgggcaggtgctggcggcccgagcgcggcccggccgctctctccaggaaaagcggaatcaatcgggtgcaaggccgactcggcccgcggggcccggcggcgggagcgctcccccggcggcccctctggctggcgcagcccgctcctcccgcgccgccgcccccgagccgagcgcga

SEQ ID NO: 9481 - RNA, 805 nt, Homo sapiens
  source 1..805: mol_type = other RNA
agggggcgggctccggcgggaccccagcgctgcaggcggtgcggctgagccagggagccccccgcgccctgcggctggatggtgaactcctcgccgtccagcaggaaggagccgctcagcccgcggcacaggctgaccgccgccagcgactcgggctccccattcacggtgccggagaagaagcagccgcgcagcccccgctcgcccccggtcgcccggccggagcccccgaggcgctcgatcttgaactcgggcgctaggaagctgtcgtcgggcgccaggcgcagcacgaagcccttgccgaaggcggacaggtggagcgcgagctcgcccgcgctgccgggcaaccgcgtgggcaccaccagctccgaggcctgccccccggctgcgggccgggccggggcgccgcgggccagcggcagcagcagcagcagcagcagcaggagcggaggccaccggggggcggcgggggcggggagcatgggggctgcggcggtggctgcgcgcaggagagggaagaagcccgccaggcgcgggcaggtgctggcggcccgagcgcggcccggccgctctctccaggaaaagcggaatcaatcgggtgcaaggccgactcggcccgcggggcccggcggcgggagcgctcccccggcggcccctctggctggcgcagcccgctcctcccgcgccgccgcccccgagccgagcgcgagcagctggccccggcccgcgtgcgcccgtcctccgcccctgcccgcgccagccccgcgcagccgcctcctgcctcctccccaccccgggaagcacc

SEQ ID NO: 9482 - RNA, 2707 nt, Homo sapiens
  source 1..2707: mol_type = other RNA
agggggcgggctccggcgggagcgcccgcgaggttaaaggggcggggggctcggccccctttctgggcggctgcgggccgtgcaggtagcgcagcagttcctccagggtggtgacttccacggcctgcccgggacagccgggcggcggtggcctcaccagcacgcggggcgcgggcccgcccgccgcgtgcccgccccgtgagcggcccggaccctccttggcgttgttcctgttctggttccactcccaggggtccccggcggcgcggaggtgcttgaccggcagctccggcgtggactcgggggtgggcaggcaggccagctccggcgggggcacgccctccggaggcggcaggaaggtggtgtagagctgcggcgtctgcaccgcgtccccgtccttggagggcggcgggggctctgggcccccaccgtggagccgggccaaactgcggagggagagagggcgcgggagccccggagtctcgatgtccttgccccgacgtcggtgggcgcggcgacaagcacaggagaccaggaggccagagactgaggcgcccagggcaaaagctgcggccacactggccaggaggagtgggatggggacggagcgggaggccgaggctgggggcaggtcccggcgcacgccataagcagaatccccagggccagactgactcccagtagctccatcttggcagtcaccatgctccatggattcctggttcccagcctgatccacatcagtcccaccagatcccctgatatccacacagcccctggagctatgccatccacagtatgggtcctgagaagccaaacagctcctctgacaggccccatgccgggcacaccggctgagagggaggtagacaatacagccagaaaaagccacaaaaagcctgtgaccctcagtgtccagctccagccctatgatccgtcgtgctgtttgggctgtccgcttcccactgcaccgggcagggctgtaggcatcaatctcttccaggaggatgggctcaggtcccccggatcgcccacctggggtcagcaccttcagcactgtcccatcattggagccaaggaacatgactgtgatgttactgtggggaccagccatgccatccacagctacttgggtcagtagggccctgctagtgagagtgagtagaggctgatgggtgacaggtggtacagcggggtccagcagcgggtgagccttgatgaaggtcaggacatcatcagggaggtctcgggaagaggagaacaaggcagctccccctactcctgcacaggatcctggcctgggtgagggaactctgtcctcagacacaggagtccaggccccatccagactcctctgctccttgaacttgccctcaaacccacgctcaatctcatccaggtagaaggcgcagacggcagagccagggatgctattggtctgggtggtgaagaccccaaagagagcagagcggccatgcaggttcacaggcccagtcaaggcctgtaaaacatcaaaatagaaagtagagtccccagggacagagcagttgagccgaagcttcaggaaggatgtccagtggcggtccaaggcccgaggcgagccgcccatgtcacgtttacatactcgggctacgcgggagaactgcaccctccccagccgagcatcctccacagagacctcgcggaagaagaagtagacatggtctccatgctccaaggcctggacaaagtgtggctctcggagccacttggagtcatacttggcggagcggagtgggggctggggcccaaggcttctgtaaactacagcatcactggcctggaaatccgcagctgtggctgagtacaggctgccctctgcaaagatggccacgttggactgggtggcatcaaaggggcatcgagcctgcccactcagttcctcaccctcctgctgcagcgaagttatcccatagctgcggcacacagggctgaatgagttcgttccacaggcaaggagcgtctgggagtcccagggaacaagaacacgaatatagttgtagcactcatccgtcagctttccccgtacagcacagttctccacatcttggcttctccatgttagatacttgttgggcaccagcccctccccttcttcttcggcttgaagatcgaaggagaaaacgtgatcccgggcagccactagcaaggtccggttcaaggtcaggaatctctgaaagtccagcccaagttctgcagccacagcatcatcctccaggccccgaaaccaggataatggggaagtaccttgaaggtcagagatcaacagagggagggggtcctggggaaaggcggcctgagtatggggaagtgagagcagcagcagcagtagcagcaagggcatgaagtggggggcacggggcatcctgtgcggggcagctcaggccccagggggtgccccctcacccataagccggccctgggttggtgactcctgtgggggcttgagggggataggaaacctctgactccaggattcgggtcagcgggatcgagatcgccgcgggcggccagcggccacgcgctgcgctgagttcgcaatccgtggttgtgctcaggcgagatgcgatgagcgtccgaattggatggtgcttgaatttgggttccagggcgctgtcgggagagccctgggtccaagtccagccgcggatccgcggaggaaaacaat

SEQ ID NO: 9483 - RNA, 4073 nt, Homo sapiens
  source 1..4073: mol_type = other RNA
agggggcgggctccggcgggagcgcccgcgaggttaaaggggcggggggctcggccccctttctgggcggctgcgggccgtgcaggtagcgcagcagttcctccagggtggtgacttccacggcctgcccgggacagccgggcggcggtggcctcaccagcacgcggggcgcgggcccgcccgccgcgtgcccgccccgtgagcggcccggaccctccttggcgttgttcctgttctggttccactcccaggggtccccggcggcgcggaggtgcttgaccggcagctccggcgtggactcgggggtgggcaggcaggccagctccggcgggggcacgccctccggaggcggcaggaaggtggtgtagagctgcggcgtctgcaccgcgtccccgtccttggagggcggcgggggctctgggcccccaccgtggagccgggccaaactgcggagggagagagggcgcgggagccccggagtctcgatgtccttgccccgacgtcggtgggcgcggcgacaagcacaggagaccaggaggccagagactgaggcgcccagggcaaaagctgcggccacactggccaggaggagtgggatggggacggagcgggaggccgaggctgggggcaggtcccggcgcacgccataagcagaatccccagggccagactgactcccagtagctccatcttggcagtcaccatgctccatggattcctggttcccagcctgatccacatcagtcccaccagatcccctgatatccacacagcccctggagctatgccatccacagtatgggtcctgagaagccaaacagctcctctgacaggccccatgccgggcacaccggctgagagggaggtagacaatacagccagaaaaagccacaaaaagcctgtgaccctcagtgtccagctccagccctatgatccgtcgtgctgtttgggctgtccgcttcccactgcaccgggcagggctgtaggcatcaatctcttccaggaggatgggctcaggtcccccggatcgcccacctggggtcagcaccttcagcactgtcccatcattggagccaaggaacatgactgtgatgttactgtggggaccagccatgccatccacagctacttgggtcagtagggccctgctagtgagagtgagtagaggctgatgggtgacaggtggtacagcggggtccagcagcgggtgagccttgatgaaggtcaggacatcatcagggaggtctcgggaagaggagaacaaggcagctccccctactcctgcacaggatcctggcctgggtgagggaactctgtcctcagacacaggagtccaggccccatccagactcctctgctccttgaacttgccctcaaacccacgctcaatctcatccaggtagaaggcgcagacggcagagccagggatgctattggtctgggtggtgaagaccccaaagagagcagagcggccatgcaggttcacaggcccagtcaaggcctgtaaaacatcaaaatagaaagtagagtccccagggacagagcagttgagccgaagcttcaggaaggatgtccagtggcggtccaaggcccgaggcgagccgcccatgtcacgtttacatactcgggctacgcgggagaactgcaccctccccagccgagcatcctccacagagacctcgcggaagaagaagtagacatggtctccatgctccaaggcctggacaaagtgtggctctcggagccacttggagtcatacttggcggagcggagtgggggctggggcccaaggcttctgtaaactacagcatcactggcctggaaatccgcagctgtggctgagtacaggctgccctctgcaaagatggccacgttggactgggtggcatcaaaggggcatcgagcctgcccactcagttcctcaccctcctgctgcagcgaagttatcccatagctgcggcacacagggctgaatgagttcgttccacaggcaaggagcgtctgggagtcccagggaacaagaacacgaatatagttgtagcactcatccgtcagctttccccgtacagcacagttctccacatcttggcttctccatgttagatacttgttgggcaccagcccctccccttcttcttcggcttgaagatcgaaggagaaaacgtgatcccgggcagccactagcaaggtccggttcaaggtcaggaatctctgaaagtccagcccaagttctgcagccacagcatcatcctccaggccccgaaaccaggataatggggaagtaccttgaaggtcagagatcaacagagggagggggtcctggggaaaggcggcctgagtatggggaagtgagagcagcagcagcagtagcagcaagggcatgaagtggggggcacggggcatcctgtgcggggcagctcaggccccagggggtgccccctcacccataagccggccctgggttggtgactcctgtgggggcttgagggggataggaaacctctgactccaggattcgggtcagcgggatcgagatcgccgcgggcggccagcggccacgcgctgcgctgagttcgcaatccgtggttgtgctcaggcgagatgcgatgagcgtccgaattggatggtgcttgaatttgggttccagggcgctgtcgggagagccctgggtccaagtccagccgcggatccgcggaggaaaacaatgcgaccgcccggggctctgggctcggccccagtggccccgcccgcctcccagccgggcccacctcctgcccgcctttgggtcgccgcgactaatcccgccctcggagggcggctagacaccgccttctcgtcacctctccgccaatagtgctgcccggggaggggcgccaggagcaccgtccacccagagggccaggccgggaggctgaactggagaccagagacagacgcgagatggagagacccacggacagtcgccgacaccgggcagaggaagaaatacatacagaagcagagacaggctggcacaggagaggctctggggagaaatttcccaagagaggaagaggagctgggaggagaaacagacaggaaacctgggagcctcgcggggctgggctgggctgtcagagcctgcgcgatccgtcctcccttcccctcctatacggcttgggcgaccttgctcccgagggcgcatcccgcatctccctgactctgcccccaactctctgttgctcctctctatgcgttgtccctctgtctccttatttctccccgtaggcctcctctggttcgtcctgacccggataaggaggcctagcatgcgcgtgggggctggaggccttggtattgcctggtaggattcttctctatgtggggctgggacaaaagacattctcaaaattctccaggaaagtgggtggcctgggagacactggcattctcagatagttttatctgactgaacacttctacccacatcttggactctggactagaggaaaggagggggaaggggtttgccactttaggccagccttaactggactgtgatcagggaggggagtatcaacaactaggctaagccccacagcgagtacacaagagacctaaacatacacacacatgtgcacacgcacatacagagaaagagagagacagagagacagatttaaggccaggtgaaccagtaagatgaacagtaactcagtaaagtcagatctaaaaaaaatagaagaagataaacagggacaatatctacacagaattaacggccgagggatcttgggtccaaggcaattcaacaaactgtcagacagttggggttgttttaaaggctggaaagaaattttcagagaaagacacctcaaaatacagaggcactgagaggttaaaagaaatctcctcagctcctagcacagggtttaggtactcagatacatgcttatggaatagattagtgagtggggattaaggtgtaattcatttaaagttttaggacccagctcaaatctcagttcaatccagtaagtattaaacacttacttgagacacaatctactacacaatccactgtgggttgtgg

SEQ ID NO: 9484 - RNA, 3965 nt, Homo sapiens
  source 1..3965: mol_type = other RNA
agggggcgggctccggcgggagcgcccgcgaggttaaaggggcggggggctcggccccctttctgggcggctgcgggccgtgcaggtagcgcagcagttcctccagggtggtgacttccacggcctgcccgggacagccgggcggcggtggcctcaccagcacgcggggcgcgggcccgcccgccgcgtgcccgccccgtgagcggcccggaccctccttggcgttgttcctgttctggttccactcccaggggtccccggcggcgcggaggtgcttgaccggcagctccggcgtggactcgggggtgggcaggcaggccagctccggcgggggcacgccctccggaggcggcaggaaggtggtgtagagctgcggcgtctgcaccgcgtccccgtccttggagggcggcgggggctctgggcccccaccgtggagccgggccaaactgcggagggagagagggcgcgggagccccggagtctcgatgtccttgccccgacgtcggtgggcgcggcgacaagcacaggagaccaggaggccagagactgaggcgcccagggcaaaagctgcggccacactggccaggaggagtgggatggggacggagcgggaggccgaggctgggggcaggtcccggcgcacgccccgagtgtgaactccaagagtggaagactggggccgggggtgggcatcactgggaggactgggggtcccaggggaagggccaggacccggaagcacataagcagaatccccagggccagactgactcccagtagctccatcttggcagtcaccatgctccatggattcctggttcccagcctgatccacatcagtcccaccagatcccctgatatccacacagcccctggagctatgccatccacagtatgggtcctgagaagccaaacagctcctctgacaggccccatgccgggcacaccggctgagagggaggtagacaatacagccagaaaaagccacaaaaagcctgtgaccctcagtgtccagctccagccctatgatccgtcgtgctgtttgggctgtccgcttcccactgcaccgggcagggctgtaggcatcaatctcttccaggaggatgggctcaggtcccccggatcgcccacctggggtcagcaccttcagcactgtcccatcattggagccaaggaacatgactgtgatgttactgtggggaccagccatgccatccacagctacttgggtcagtagggccctgctagtgagagtgagtagaggctgatgggtgacaggtggtacagcggggtccagcagcgggtgagccttgatgaaggtcaggacatcatcagggaggtctcgggaagaggagaacaaggcagctccccctactcctgcacaggatcctggcctgggtgagggaactctgtcctcagacacaggagtccaggccccatccagactcctctgctccttgaacttgccctcaaacccacgctcaatctcatccaggtagaaggcgcagacggcagagccagggatgctattggtctgggtggtgaagaccccaaagagagcagagcggccatgcaggttcacaggcccagtcaaggcctgtaaaacatcaaaatagaaagtagagtccccagggacagagcagttgagccgaagcttcaggaaggatgtccagtggcggtccaaggcccgaggcgagccgcccatgtcacgtttacatactcgggctacgcgggagaactgcaccctccccagccgagcatcctccacagagacctcgcggaagaagaagtagacatggtctccatgctccaaggcctggacaaagtgtggctctcggagccacttggagtcatacttggcggagcggagtgggggctggggcccaaggcttctgtaaactacagcatcactggcctggaaatccgcagctgtggctgagtacaggctgccctctgcaaagatggccacgttggactgggtggcatcaaaggggcatcgagcctgcccactcagttcctcaccctcctgctgcagcgaagttatcccatagctgcggcacacagggctgaatgagttcgttccacaggcaaggagcgtctgggagtcccagggaacaagaacacgaatatagttgtagcactcatccgtcagctttccccgtacagcacagttctccacatcttggcttctccatgttagatacttgttgggcaccagcccctccccttcttcttcggcttgaagatcgaaggagaaaacgtgatcccgggcagccactagcaaggtccggttcaaggtcaggaatctctgaaagtccagcccaagttctgcagccacagcatcatcctccaggccccgaaaccaggataatggggaagtaccttgaaggtcagagatcaacagagggagggggtcctggggaaaggcggcctgagtatggggaagtgagagcagcagcagcagtagcagcaagggcatgaagtggggggcacggggcatcctgtgcggggcagctcaggccccagggggtgccccctcacccataagccggccctgggttggtgactcctgtgggggcttgagggggataggaaacctctgacctttaagagggcttcttgtagctgtttctgggaagcagcatctggtcagctcctcaactcctggcctggagaaaagatcactctgccctggaagaatccgagctgcttcacacaccccatctgaagcacatgggagagacctggccgactctcccctttccagatcctcccgttgctgggaagaggaaacagcccttctctctcctggccccgaagccacctctggggaatggctggggtcacagccagagtctaggagagctgtggaagggatggagaaggggagactgggctggggacaatagcaggaagcctttgggctggtcgcccgccccagtccaccttcctcagagggagcagggtcgcgccaaggagcctgtggaaccggagctttcctttctccaagccatttcccccactcttagctcttagccccacactcagcacctaccctccttcccacccaacccccaaccaggacaatccaggtgtctaaagcctcgaaaagaggtgggcctagggccaggggctcgacctgtctccccctcaccggatccggggctccgaggaggggccggtagcagagtctgggccgggaccgggtcccagagccacgttagcgagaggaggggctggaggggcctgcaggcgcagacgaagaggggataggagcgggggttggggagcggaggcgggtctcccaggccagggaaacagggccagaggctgagaaccgacgagggcgggcctgaggccggcgctcagtggggaccgtgggctcaggaggcagttgccagctcggatgtcctccttgggagacctcagtctaacaaagccccgggccgagcgggctgaaggaaggagataggcgctgggaccgatgttgctcgagggccccattcgccgcctctttgcacgagccaacccttcagagggtgctcagattccggcttgcacaaggacagaggagcacccgtgacacaaagtccggaacgatgcgtccctcttcccatcccttcaggggcgtcaggagggtctagttctccgtgggtctcggagccctagtttccttgctgggaaagcaaggggccaggttttccacgctctctacggagcgcgcctcaaataatcccttttcgcgcttcccagtccagcgggatgcgactcgacgaaagcccaattgaacgaggtgcccagactctgctctcaccagtacagttacggggctcggccactgtccctccttcctccctgcaccccaatttcgttgaccctctccgtcagccaggcacaccgggcgccgacacctccctggtcccctagcgcttcagaagcttgccccccgccggccgcgccctcct

SEQ ID NO: 9485 - RNA, 3975 nt, Homo sapiens
  source 1..3975: mol_type = other RNA
agggggcgggctccggcgggagcgcccgcgaggttaaaggggcggggggctcggccccctttctgggcggctgcgggccgtgcaggtagcgcagcagttcctccagggtggtgacttccacggcctgcccgggacagccgggcggcggtggcctcaccagcacgcggggcgcgggcccgcccgccgcgtgcccgccccgtgagcggcccggaccctccttggcgttgttcctgttctggttccactcccaggggtccccggcggcgcggaggtgcttgaccggcagctccggcgtggactcgggggtgggcaggcaggccagctccggcgggggcacgccctccggaggcggcaggaaggtggtgtagagctgcggcgtctgcaccgcgtccccgtccttggagggcggcgggggctctgggcccccaccgtggagccgggccaaactgcggagggagagagggcgcgggagccccggagtctcgatgtccttgccccgacgtcggtgggcgcggcgacaagcacaggagaccaggaggccagagactgaggcgcccagggcaaaagctgcggccacactggccaggaggagtgggatggggacggagcgggaggccgaggctgggggcaggtcccggcgcacgccccgagtgtgaactccaagagtggaagactggggccgggggtgggcatcactgggaggactgggggtcccaggggaagggccaggacccggaagcacataagcagaatccccagggccagactgactcccagtagctccatcttggcagtcaccatgctccatggattcctggttcccagcctgatccacatcagtcccaccagatcccctgatatccacacagcccctggagctatgccatccacagtatgggtcctgagaagccaaacagctcctctgacaggccccatgccgggcacaccggctgagagggaggtagacaatacagccagaaaaagccacaaaaagcctgtgaccctcagtgtccagctccagccctatgatccgtcgtgctgtttgggctgtccgcttcccactgcaccgggcagggctgtaggcatcaatctcttccaggaggatgggctcaggtcccccggatcgcccacctggggtcagcaccttcagcactgtcccatcattggagccaaggaacatgactgtgatgttactgtggggaccagccatgccatccacagctacttgggtcagtagggccctgctagtgagagtgagtagaggctgatgggtgacaggtggtacagcggggtccagcagcgggtgagccttgatgaaggtcaggacatcatcagggaggtctcgggaagaggagaacaaggcagctccccctactcctgcacaggatcctggcctgggtgagggaactctgtcctcagacacaggagtccaggccccatccagactcctctgctccttgaacttgccctcaaacccacgctcaatctcatccaggtagaaggcgcagacggcagagccagggatgctattggtctgggtggtgaagaccccaaagagagcagagcggccatgcaggttcacaggcccagtcaaggcctgtaaaacatcaaaatagaaagtagagtccccagggacagagcagttgagccgaagcttcaggaaggatgtccagtggcggtccaaggcccgaggcgagccgcccatgtcacgtttacatactcgggctacgcgggagaactgcaccctccccagccgagcatcctccacagagacctcgcggaagaagaagtagacatggtctccatgctccaaggcctggacaaagtgtggctctcggagccacttggagtcatacttggcggagcggagtgggggctggggcccaaggcttctgtaaactacagcatcactggcctggaaatccgcagctgtggctgagtacaggctgccctctgcaaagatggccacgttggactgggtggcatcaaaggggcatcgagcctgcccactcagttcctcaccctcctgctgcagcgaagttatcccatagctgcggcacacagggctgaatgagttcgttccacaggcaaggagcgtctgggagtcccagggaacaagaacacgaatatagttgtagcactcatccgtcagctttccccgtacagcacagttctccacatcttggcttctccatgttagatacttgttgggcaccagcccctccccttcttcttcggcttgaagatcgaaggagaaaacgtgatcccgggcagccactagcaaggtccggttcaaggtcaggaatctctgaaagtccagcccaagttctgcagccacagcatcatcctccaggccccgaaaccaggataatggggaagtaccttgaaggtcagagatcaacagagggagggggtcctggggaaaggcggcctgagtatggggaagtgagagcagcagcagcagtagcagcaagggcatgaagtggggggcacggggcatcctgtgcggggcagctcaggccccagggggtgccccctcacccataagccggccctgggttggtgactcctgtgggggcttgagggggataggaaacctctgactatgatacacctttaagagggcttcttgtagctgtttctgggaagcagcatctggtcagctcctcaactcctggcctggagaaaagatcactctgccctggaagaatccgagctgcttcacacaccccatctgaagcacatgggagagacctggccgactctcccctttccagatcctcccgttgctgggaagaggaaacagcccttctctctcctggccccgaagccacctctggggaatggctggggtcacagccagagtctaggagagctgtggaagggatggagaaggggagactgggctggggacaatagcaggaagcctttgggctggtcgcccgccccagtccaccttcctcagagggagcagggtcgcgccaaggagcctgtggaaccggagctttcctttctccaagccatttcccccactcttagctcttagccccacactcagcacctaccctccttcccacccaacccccaaccaggacaatccaggtgtctaaagcctcgaaaagaggtgggcctagggccaggggctcgacctgtctccccctcaccggatccggggctccgaggaggggccggtagcagagtctgggccgggaccgggtcccagagccacgttagcgagaggaggggctggaggggcctgcaggcgcagacgaagaggggataggagcgggggttggggagcggaggcgggtctcccaggccagggaaacagggccagaggctgagaaccgacgagggcgggcctgaggccggcgctcagtggggaccgtgggctcaggaggcagttgccagctcggatgtcctccttgggagacctcagtctaacaaagccccgggccgagcgggctgaaggaaggagataggcgctgggaccgatgttgctcgagggccccattcgccgcctctttgcacgagccaacccttcagagggtgctcagattccggcttgcacaaggacagaggagcacccgtgacacaaagtccggaacgatgcgtccctcttcccatcccttcaggggcgtcaggagggtctagttctccgtgggtctcggagccctagtttccttgctgggaaagcaaggggccaggttttccacgctctctacggagcgcgcctcaaataatcccttttcgcgcttcccagtccagcgggatgcgactcgacgaaagcccaattgaacgaggtgcccagactctgctctcaccagtacagttacggggctcggccactgtccctccttcctccctgcaccccaatttcgttgaccctctccgtcagccaggcacaccgggcgccgacacctccctggtcccctagcgcttcagaagcttgccccccgccggccgcgccctcct

SEQ ID NO: 9486 - RNA, 2803 nt, Homo sapiens
  source 1..2803: mol_type = other RNA
agggggcgggctccggcgggagcgcccgcgaggttaaaggggcggggggctcggccccctttctgggcggctgcgggccgtgcaggtagcgcagcagttcctccagggtggtgacttccacggcctgcccgggacagccgggcggcggtggcctcaccagcacgcggggcgcgggcccgcccgccgcgtgcccgccccgtgagcggcccggaccctccttggcgttgttcctgttctggttccactcccaggggtccccggcggcgcggaggtgcttgaccggcagctccggcgtggactcgggggtgggcaggcaggccagctccggcgggggcacgccctccggaggcggcaggaaggtggtgtagagctgcggcgtctgcaccgcgtccccgtccttggagggcggcgggggctctgggcccccaccgtggagccgggccaaactgcggagggagagagggcgcgggagccccggagtctcgatgtccttgccccgacgtcggtgggcgcggcgacaagcacaggagaccaggaggccagagactgaggcgcccagggcaaaagctgcggccacactggccaggaggagtgggatggggacggagcgggaggccgaggctgggggcaggtcccggcgcacgccccgagtgtgaactccaagagtggaagactggggccgggggtgggcatcactgggaggactgggggtcccaggggaagggccaggacccggaagcacataagcagaatccccagggccagactgactcccagtagctccatcttggcagtcaccatgctccatggattcctggttcccagcctgatccacatcagtcccaccagatcccctgatatccacacagcccctggagctatgccatccacagtatgggtcctgagaagccaaacagctcctctgacaggccccatgccgggcacaccggctgagagggaggtagacaatacagccagaaaaagccacaaaaagcctgtgaccctcagtgtccagctccagccctatgatccgtcgtgctgtttgggctgtccgcttcccactgcaccgggcagggctgtaggcatcaatctcttccaggaggatgggctcaggtcccccggatcgcccacctggggtcagcaccttcagcactgtcccatcattggagccaaggaacatgactgtgatgttactgtggggaccagccatgccatccacagctacttgggtcagtagggccctgctagtgagagtgagtagaggctgatgggtgacaggtggtacagcggggtccagcagcgggtgagccttgatgaaggtcaggacatcatcagggaggtctcgggaagaggagaacaaggcagctccccctactcctgcacaggatcctggcctgggtgagggaactctgtcctcagacacaggagtccaggccccatccagactcctctgctccttgaacttgccctcaaacccacgctcaatctcatccaggtagaaggcgcagacggcagagccagggatgctattggtctgggtggtgaagaccccaaagagagcagagcggccatgcaggttcacaggcccagtcaaggcctgtaaaacatcaaaatagaaagtagagtccccagggacagagcagttgagccgaagcttcaggaaggatgtccagtggcggtccaaggcccgaggcgagccgcccatgtcacgtttacatactcgggctacgcgggagaactgcaccctccccagccgagcatcctccacagagacctcgcggaagaagaagtagacatggtctccatgctccaaggcctggacaaagtgtggctctcggagccacttggagtcatacttggcggagcggagtgggggctggggcccaaggcttctgtaaactacagcatcactggcctggaaatccgcagctgtggctgagtacaggctgccctctgcaaagatggccacgttggactgggtggcatcaaaggggcatcgagcctgcccactcagttcctcaccctcctgctgcagcgaagttatcccatagctgcggcacacagggctgaatgagttcgttccacaggcaaggagcgtctgggagtcccagggaacaagaacacgaatatagttgtagcactcatccgtcagctttccccgtacagcacagttctccacatcttggcttctccatgttagatacttgttgggcaccagcccctccccttcttcttcggcttgaagatcgaaggagaaaacgtgatcccgggcagccactagcaaggtccggttcaaggtcaggaatctctgaaagtccagcccaagttctgcagccacagcatcatcctccaggccccgaaaccaggataatggggaagtaccttgaaggtcagagatcaacagagggagggggtcctggggaaaggcggcctgagtatggggaagtgagagcagcagcagcagtagcagcaagggcatgaagtggggggcacggggcatcctgtgcggggcagctcaggccccagggggtgccccctcacccataagccggccctgggttggtgactcctgtgggggcttgagggggataggaaacctctgactccaggattcgggtcagcgggatcgagatcgccgcgggcggccagcggccacgcgctgcgctgagttcgcaatccgtggttgtgctcaggcgagatgcgatgagcgtccgaattggatggtgcttgaatttgggttccagggcgctgtcgggagagccctgggtccaagtccagccgcggatccgcggaggaaaacaat

SEQ ID NO: 9487 - RNA, 4169 nt, Homo sapiens
  source 1..4169: mol_type = other RNA
agggggcgggctccggcgggagcgcccgcgaggttaaaggggcggggggctcggccccctttctgggcggctgcgggccgtgcaggtagcgcagcagttcctccagggtggtgacttccacggcctgcccgggacagccgggcggcggtggcctcaccagcacgcggggcgcgggcccgcccgccgcgtgcccgccccgtgagcggcccggaccctccttggcgttgttcctgttctggttccactcccaggggtccccggcggcgcggaggtgcttgaccggcagctccggcgtggactcgggggtgggcaggcaggccagctccggcgggggcacgccctccggaggcggcaggaaggtggtgtagagctgcggcgtctgcaccgcgtccccgtccttggagggcggcgggggctctgggcccccaccgtggagccgggccaaactgcggagggagagagggcgcgggagccccggagtctcgatgtccttgccccgacgtcggtgggcgcggcgacaagcacaggagaccaggaggccagagactgaggcgcccagggcaaaagctgcggccacactggccaggaggagtgggatggggacggagcgggaggccgaggctgggggcaggtcccggcgcacgccccgagtgtgaactccaagagtggaagactggggccgggggtgggcatcactgggaggactgggggtcccaggggaagggccaggacccggaagcacataagcagaatccccagggccagactgactcccagtagctccatcttggcagtcaccatgctccatggattcctggttcccagcctgatccacatcagtcccaccagatcccctgatatccacacagcccctggagctatgccatccacagtatgggtcctgagaagccaaacagctcctctgacaggccccatgccgggcacaccggctgagagggaggtagacaatacagccagaaaaagccacaaaaagcctgtgaccctcagtgtccagctccagccctatgatccgtcgtgctgtttgggctgtccgcttcccactgcaccgggcagggctgtaggcatcaatctcttccaggaggatgggctcaggtcccccggatcgcccacctggggtcagcaccttcagcactgtcccatcattggagccaaggaacatgactgtgatgttactgtggggaccagccatgccatccacagctacttgggtcagtagggccctgctagtgagagtgagtagaggctgatgggtgacaggtggtacagcggggtccagcagcgggtgagccttgatgaaggtcaggacatcatcagggaggtctcgggaagaggagaacaaggcagctccccctactcctgcacaggatcctggcctgggtgagggaactctgtcctcagacacaggagtccaggccccatccagactcctctgctccttgaacttgccctcaaacccacgctcaatctcatccaggtagaaggcgcagacggcagagccagggatgctattggtctgggtggtgaagaccccaaagagagcagagcggccatgcaggttcacaggcccagtcaaggcctgtaaaacatcaaaatagaaagtagagtccccagggacagagcagttgagccgaagcttcaggaaggatgtccagtggcggtccaaggcccgaggcgagccgcccatgtcacgtttacatactcgggctacgcgggagaactgcaccctccccagccgagcatcctccacagagacctcgcggaagaagaagtagacatggtctccatgctccaaggcctggacaaagtgtggctctcggagccacttggagtcatacttggcggagcggagtgggggctggggcccaaggcttctgtaaactacagcatcactggcctggaaatccgcagctgtggctgagtacaggctgccctctgcaaagatggccacgttggactgggtggcatcaaaggggcatcgagcctgcccactcagttcctcaccctcctgctgcagcgaagttatcccatagctgcggcacacagggctgaatgagttcgttccacaggcaaggagcgtctgggagtcccagggaacaagaacacgaatatagttgtagcactcatccgtcagctttccccgtacagcacagttctccacatcttggcttctccatgttagatacttgttgggcaccagcccctccccttcttcttcggcttgaagatcgaaggagaaaacgtgatcccgggcagccactagcaaggtccggttcaaggtcaggaatctctgaaagtccagcccaagttctgcagccacagcatcatcctccaggccccgaaaccaggataatggggaagtaccttgaaggtcagagatcaacagagggagggggtcctggggaaaggcggcctgagtatggggaagtgagagcagcagcagcagtagcagcaagggcatgaagtggggggcacggggcatcctgtgcggggcagctcaggccccagggggtgccccctcacccataagccggccctgggttggtgactcctgtgggggcttgagggggataggaaacctctgactccaggattcgggtcagcgggatcgagatcgccgcgggcggccagcggccacgcgctgcgctgagttcgcaatccgtggttgtgctcaggcgagatgcgatgagcgtccgaattggatggtgcttgaatttgggttccagggcgctgtcgggagagccctgggtccaagtccagccgcggatccgcggaggaaaacaatgcgaccgcccggggctctgggctcggccccagtggccccgcccgcctcccagccgggcccacctcctgcccgcctttgggtcgccgcgactaatcccgccctcggagggcggctagacaccgccttctcgtcacctctccgccaatagtgctgcccggggaggggcgccaggagcaccgtccacccagagggccaggccgggaggctgaactggagaccagagacagacgcgagatggagagacccacggacagtcgccgacaccgggcagaggaagaaatacatacagaagcagagacaggctggcacaggagaggctctggggagaaatttcccaagagaggaagaggagctgggaggagaaacagacaggaaacctgggagcctcgcggggctgggctgggctgtcagagcctgcgcgatccgtcctcccttcccctcctatacggcttgggcgaccttgctcccgagggcgcatcccgcatctccctgactctgcccccaactctctgttgctcctctctatgcgttgtccctctgtctccttatttctccccgtaggcctcctctggttcgtcctgacccggataaggaggcctagcatgcgcgtgggggctggaggccttggtattgcctggtaggattcttctctatgtggggctgggacaaaagacattctcaaaattctccaggaaagtgggtggcctgggagacactggcattctcagatagttttatctgactgaacacttctacccacatcttggactctggactagaggaaaggagggggaaggggtttgccactttaggccagccttaactggactgtgatcagggaggggagtatcaacaactaggctaagccccacagcgagtacacaagagacctaaacatacacacacatgtgcacacgcacatacagagaaagagagagacagagagacagatttaaggccaggtgaaccagtaagatgaacagtaactcagtaaagtcagatctaaaaaaaatagaagaagataaacagggacaatatctacacagaattaacggccgagggatcttgggtccaaggcaattcaacaaactgtcagacagttggggttgttttaaaggctggaaagaaattttcagagaaagacacctcaaaatacagaggcactgagaggttaaaagaaatctcctcagctcctagcacagggtttaggtactcagatacatgcttatggaatagattagtgagtggggattaaggtgtaattcatttaaagttttaggacccagctcaaatctcagttcaatccagtaagtattaaacacttacttgagacacaatctactacacaatccactgtgggttgtgg

SEQ ID NO: 9488 - RNA, 2840 nt, Homo sapiens
  source 1..2840: mol_type = other RNA
agggggcgggctccggcgggagcgcccgcgaggttaaaggggcggggggctcggccccctttctgggcggctgcgggccgtgcaggtagcgcagcagttcctccagggtggtgacttccacggcctgcccgggacagccgggcggcggtggcctcaccagcacgcggggcgcgggcccgcccgccgcgtgcccgccccgtgagcggcccggaccctccttggcgttgttcctgttctggttccactcccaggggtccccggcggcgcggaggtgcttgaccggcagctccggcgtggactcgggggtgggcaggcaggccagctccggcgggggcacgccctccggaggcggcaggaaggtggtgtagagctgcggcgtctgcaccgcgtccccgtccttggagggcggcgggggctctgggcccccaccgtggagccgggccaaactgcggagggagagagggcgcgggagccccggagtctcgatgtccttgccccgacgtcggtgggcgcggcgacaagcacaggagaccaggaggccagagactgaggcgcccagggcaaaagctgcggccacactggccaggaggagtgggatggggacggagcgggaggccgaggctgggggcaggtcccggcgcacgccccgagtgtgaactccaagagtggaagactggggccgggggtgggcatcactgggaggactgggggtcccaggggaagggccaggacccggaagcacataagcagaatccccagggccagactgactcccagtagctccatcttggcagtcaccatgctccatggattcctggttcccagcctgatccacatcagtcccaccagatcccctgatatccacacagcccctggagctatgccatccacagtatgggtcctgagaagccaaacagctcctctgacaggccccatgccgggcacaccggctgagagggaggtagacaatacagccagaaaaagccacaaaaagcctgtgaccctcagtgtccagctccagccctatgatccgtcgtgctgtttgggctgtccgcttcccactgcaccgggcagggctgtaggcatcaatctcttccaggaggatgggctcaggtcccccggatcgcccacctggggtcagcaccttcagcactgtcccatcattggagccaaggaacatgactgtgatgttactgtggggaccagccatgccatccacagctacttgggtcagtagggccctgctagtgagagtgagtagaggctgatgggtgacaggtggtacagcggggtccagcagcgggtgagccttgatgaaggtcaggacatcatcagggaggtctcgggaagaggagaacaaggcagctccccctactcctgcacaggatcctggcctgggtgagggaactctgtcctcagacacaggagtccaggccccatccagactcctctgctccttgaacttgccctcaaacccacgctcaatctcatccaggtagaaggcgcagacggcagagccagggatgctattggtctgggtggtgaagaccccaaagagagcagagcggccatgcaggttcacaggcccagtcaaggcctgtaaaacatcaaaatagaaagtagagtccccagggacagagcagttgagccgaagcttcaggaaggatgtccagtggcggtccaaggcccgaggcgagccgcccatgtcacgtttacatactcgggctacgcgggagaactgcaccctccccagccgagcatcctccacagagacctcgcggaagaagaagtagacatggtctccatgctccaaggcctggacaaagtgtggctctcggagccacttggagtcatacttggcggagcggagtgggggctggggcccaaggcttctgtaaactacagcatcactggcctggaaatccgcagctgtggctgagtacaggctgccctctgcaaagatggccacgttggactgggtggcatcaaaggggcatcgagcctgcccactcagttcctcaccctcctgctgcagcgaagttatcccatagctgcggcacacagggctgaatgagttcgttccacaggcaaggagcgtctgggagtcccagggaacaagaacacgaatatagttgtagcactcatccgtcagctttccccgtacagcacagttctccacatcttggcttctccatgttagatacttgttgggcaccagcccctccccttcttcttcggcttgaagatcgaaggagaaaacgtgatcccgggcagccactagcaaggtccggttcaaggtcaggaatctctgaaagtccagcccaagttctgcagccacagcatcatcctccaggccccgaaaccaggataatggggaagtaccttgaaggtcagagatcaacagagggagggggtcctggggaaaggcggcctgagtatggggaagtgagagcagcagcagcagtagcagcaagggcatgaagtggggggcacggggcatcctgtgcggggcagctcaggccccagggggtgccccctcacccataagccggccctgggttggtgactcctgtgggggcttgagggggataggaaacctctgacttgctccaggattcgggtcagcgggatcgagatcgccgcgggcggccagcggccacgcgctgcgctgagttcgcaatccgtggttgtgctcaggcgagatgcgatgagcgtccgaattggatggtgcttgaatttgggttccagggcgctgtcgggagagccctgggtccaagtccagccgcggatccgcggaggaaaacaatgcgaccgcccggggctctgggctcggccccagt

SEQ ID NO: 9489 - RNA, 2683 nt, Homo sapiens
  source 1..2683: mol_type = other RNA
agggggcgggctccggcgggagcgcccgcgaggttaaaggggcggggggctcggccccctttctgggcggctgcgggccgtgcaggtagcgcagcagttcctccagggtggtgacttccacggcctgcccgggacagccgggcggcggtggcctcaccagcacgcggggcgcgggcccgcccgccgcgtgcccgccccgtgagcggcccggaccctccttggcgttgttcctgttctggttccactcccaggggtccccggcggcgcggaggtgcttgaccggcagctccggcgtggactcgggggtgggcaggcaggccagctccggcgggggcacgccctccggaggcggcaggaaggtggtgtagagctgcggcgtctgcaccgcgtccccgtccttggagggcggcgggggctctgggcccccaccgtggagccgggccaaactgcggagggagagagggcgcgggagccccggagtctcgatgtccttgccccgacgtcggtgggcgcggcgacaagcacaggagaccaggaggccagagactgaggcgcccagggcaaaagctgcggccacactggccaggaggagtgggatggggacggagcgggaggccgaggctgggggcaggtcccggcgcacgccccgagtgtgaactccaagagtggaagactggggccgggggtgggcatcactgggaggactgggggtcccaggggaagggccaggacccggaagcacataagcagaatccccagggccagactgactcccagtagctccatcttggcagtcaccatgctccatggattcctggttcccagcctgatccacatcagtcccaccagatcccctgatatccacacagcccctggagctatgccatccacagtatgggtcctgagaagccaaacagctcctctgacaggccccatgccgggcacaccggctgagagggaggtagacaatacagccagaaaaagccacaaaaagcctgtgaccctcagtgtccagctccagccctatgatccgtcgtgctgtttgggctgtccgcttcccactgcaccgggcagggctgtaggcatcaatctcttccaggaggatgggctcaggtcccccggatcgcccacctggggtcagcaccttcagcactgtcccatcattggagccaaggaacatgactgtgatgttactgtggggaccagccatgccatccacagctacttgggtcagtagggccctgctagtgagagtgagtagaggctgatgggtgacaggtggtacagcggggtccagcagcgggtgagccttgatgaaggtcaggacatcatcagggaggtctcgggaagaggagaacaaggcagctccccctactcctgcacaggatcctggcctgggtgagggaactctgtcctcagacacaggagtccaggccccatccagactcctctgctccttgaacttgccctcaaacccacgctcaatctcatccaggtagaaggcgcagacggcagagccagggatgctattggtctgggtggtgaagaccccaaagagagcagagcggccatgcaggttcacaggcccagtcaaggcctgtaaaacatcaaaatagaaagtagagtccccagggacagagcagttgagccgaagcttcaggaaggatgtccagtggcggtccaaggcccgaggcgagccgcccatgtcacgtttacatactcgggctacgcgggagaactgcaccctccccagccgagcatcctccacagagacctcgcggaagaagaagtagacatggtctccatgctccaaggcctggacaaagtgtggctctgcaaagatggccacgttggactgggtggcatcaaaggggcatcgagcctgcccactcagttcctcaccctcctgctgcagcgaagttatcccatagctgcggcacacagggctgaatgagttcgttccacaggcaaggagcgtctgggagtcccagggaacaagaacacgaatatagttgtagcactcatccgtcagctttccccgtacagcacagttctccacatcttggcttctccatgttagatacttgttgggcaccagcccctccccttcttcttcggcttgaagatcgaaggagaaaacgtgatcccgggcagccactagcaaggtccggttcaaggtcaggaatctctgaaagtccagcccaagttctgcagccacagcatcatcctccaggccccgaaaccaggataatggggaagtaccttgaaggtcagagatcaacagagggagggggtcctggggaaaggcggcctgagtatggggaagtgagagcagcagcagcagtagcagcaagggcatgaagtggggggcacggggcatcctgtgcggggcagctcaggccccagggggtgccccctcacccataagccggccctgggttggtgactcctgtgggggcttgagggggataggaaacctctgactccaggattcgggtcagcgggatcgagatcgccgcgggcggccagcggccacgcgctgcgctgagttcgcaatccgtggttgtgctcaggcgagatgcgatgagcgtccgaattggatggtgcttgaatttgggttccagggcgctgtcgggagagccctgggtccaagtccagccgcggatccgcggaggaaaacaat

SEQ ID NO: 9490 - RNA, 4049 nt, Homo sapiens
  source 1..4049: mol_type = other RNA
agggggcgggctccggcgggagcgcccgcgaggttaaaggggcggggggctcggccccctttctgggcggctgcgggccgtgcaggtagcgcagcagttcctccagggtggtgacttccacggcctgcccgggacagccgggcggcggtggcctcaccagcacgcggggcgcgggcccgcccgccgcgtgcccgccccgtgagcggcccggaccctccttggcgttgttcctgttctggttccactcccaggggtccccggcggcgcggaggtgcttgaccggcagctccggcgtggactcgggggtgggcaggcaggccagctccggcgggggcacgccctccggaggcggcaggaaggtggtgtagagctgcggcgtctgcaccgcgtccccgtccttggagggcggcgggggctctgggcccccaccgtggagccgggccaaactgcggagggagagagggcgcgggagccccggagtctcgatgtccttgccccgacgtcggtgggcgcggcgacaagcacaggagaccaggaggccagagactgaggcgcccagggcaaaagctgcggccacactggccaggaggagtgggatggggacggagcgggaggccgaggctgggggcaggtcccggcgcacgccccgagtgtgaactccaagagtggaagactggggccgggggtgggcatcactgggaggactgggggtcccaggggaagggccaggacccggaagcacataagcagaatccccagggccagactgactcccagtagctccatcttggcagtcaccatgctccatggattcctggttcccagcctgatccacatcagtcccaccagatcccctgatatccacacagcccctggagctatgccatccacagtatgggtcctgagaagccaaacagctcctctgacaggccccatgccgggcacaccggctgagagggaggtagacaatacagccagaaaaagccacaaaaagcctgtgaccctcagtgtccagctccagccctatgatccgtcgtgctgtttgggctgtccgcttcccactgcaccgggcagggctgtaggcatcaatctcttccaggaggatgggctcaggtcccccggatcgcccacctggggtcagcaccttcagcactgtcccatcattggagccaaggaacatgactgtgatgttactgtggggaccagccatgccatccacagctacttgggtcagtagggccctgctagtgagagtgagtagaggctgatgggtgacaggtggtacagcggggtccagcagcgggtgagccttgatgaaggtcaggacatcatcagggaggtctcgggaagaggagaacaaggcagctccccctactcctgcacaggatcctggcctgggtgagggaactctgtcctcagacacaggagtccaggccccatccagactcctctgctccttgaacttgccctcaaacccacgctcaatctcatccaggtagaaggcgcagacggcagagccagggatgctattggtctgggtggtgaagaccccaaagagagcagagcggccatgcaggttcacaggcccagtcaaggcctgtaaaacatcaaaatagaaagtagagtccccagggacagagcagttgagccgaagcttcaggaaggatgtccagtggcggtccaaggcccgaggcgagccgcccatgtcacgtttacatactcgggctacgcgggagaactgcaccctccccagccgagcatcctccacagagacctcgcggaagaagaagtagacatggtctccatgctccaaggcctggacaaagtgtggctctgcaaagatggccacgttggactgggtggcatcaaaggggcatcgagcctgcccactcagttcctcaccctcctgctgcagcgaagttatcccatagctgcggcacacagggctgaatgagttcgttccacaggcaaggagcgtctgggagtcccagggaacaagaacacgaatatagttgtagcactcatccgtcagctttccccgtacagcacagttctccacatcttggcttctccatgttagatacttgttgggcaccagcccctccccttcttcttcggcttgaagatcgaaggagaaaacgtgatcccgggcagccactagcaaggtccggttcaaggtcaggaatctctgaaagtccagcccaagttctgcagccacagcatcatcctccaggccccgaaaccaggataatggggaagtaccttgaaggtcagagatcaacagagggagggggtcctggggaaaggcggcctgagtatggggaagtgagagcagcagcagcagtagcagcaagggcatgaagtggggggcacggggcatcctgtgcggggcagctcaggccccagggggtgccccctcacccataagccggccctgggttggtgactcctgtgggggcttgagggggataggaaacctctgactccaggattcgggtcagcgggatcgagatcgccgcgggcggccagcggccacgcgctgcgctgagttcgcaatccgtggttgtgctcaggcgagatgcgatgagcgtccgaattggatggtgcttgaatttgggttccagggcgctgtcgggagagccctgggtccaagtccagccgcggatccgcggaggaaaacaatgcgaccgcccggggctctgggctcggccccagtggccccgcccgcctcccagccgggcccacctcctgcccgcctttgggtcgccgcgactaatcccgccctcggagggcggctagacaccgccttctcgtcacctctccgccaatagtgctgcccggggaggggcgccaggagcaccgtccacccagagggccaggccgggaggctgaactggagaccagagacagacgcgagatggagagacccacggacagtcgccgacaccgggcagaggaagaaatacatacagaagcagagacaggctggcacaggagaggctctggggagaaatttcccaagagaggaagaggagctgggaggagaaacagacaggaaacctgggagcctcgcggggctgggctgggctgtcagagcctgcgcgatccgtcctcccttcccctcctatacggcttgggcgaccttgctcccgagggcgcatcccgcatctccctgactctgcccccaactctctgttgctcctctctatgcgttgtccctctgtctccttatttctccccgtaggcctcctctggttcgtcctgacccggataaggaggcctagcatgcgcgtgggggctggaggccttggtattgcctggtaggattcttctctatgtggggctgggacaaaagacattctcaaaattctccaggaaagtgggtggcctgggagacactggcattctcagatagttttatctgactgaacacttctacccacatcttggactctggactagaggaaaggagggggaaggggtttgccactttaggccagccttaactggactgtgatcagggaggggagtatcaacaactaggctaagccccacagcgagtacacaagagacctaaacatacacacacatgtgcacacgcacatacagagaaagagagagacagagagacagatttaaggccaggtgaaccagtaagatgaacagtaactcagtaaagtcagatctaaaaaaaatagaagaagataaacagggacaatatctacacagaattaacggccgagggatcttgggtccaaggcaattcaacaaactgtcagacagttggggttgttttaaaggctggaaagaaattttcagagaaagacacctcaaaatacagaggcactgagaggttaaaagaaatctcctcagctcctagcacagggtttaggtactcagatacatgcttatggaatagattagtgagtggggattaaggtgtaattcatttaaagttttaggacccagctcaaatctcagttcaatccagtaagtattaaacacttacttgagacacaatctactacacaatccactgtgggttgtgg

SEQ ID NO: 9491 - RNA, 1948 nt, Homo sapiens
  source 1..1948: mol_type = other RNA
agggggcgggctccggcgggagcgcccgcgaggttaaaggggcggggggctcggccccctttctgggcggctgcgggccgtgcaggtagcgcagcagttcctccagggtggtgacttccacggcctgcccgggacagccgggcggcggtggcctcaccagcacgcggggcgcgggcccgcccgccgcgtgcccgccccgtgagcggcccggaccctccttggcgttgttcctgttctggttccactcccaggggtccccggcggcgcggaggtgcttgaccggcagctccggcgtggactcgggggtgggcaggcaggccagctccggcgggggcacgccctccggaggcggcaggaaggtggtgtagagctgcggcgtctgcaccgcgtccccgtccttggagggcggcgggggctctgggcccccaccgtggagccgggccaaactgcggagggagagagggcgcgggagccccggagtctcgatgtccttgccccgacgtcggtgggcgcggcgacaagcacaggagaccaggaggccagagactgaggcgcccagggcaaaagctgcggccacactggccaggaggagtgggatggggacggagcgggaggccgaggctgggggcaggtcccggcgcacgccccgagtgtgaactccaagagtggaagactggggccgggggtgggcatcactgggaggactgggggtcccaggggaagggccaggacccggaagcacataagcagaatccccagggccagactgactcccagtagctccatcttggcagtcaccatgctccatggattcctggttcccagcctgatccacatcagtcccaccagatcccctgatatccacacagcccctggagctatgccatccacagtatgggtcctgagaagccaaacagctcctctgacaggccccatgccgggcacaccggctgagagggaggtagacaatacagccagaaaaagccacaaaaagcctgtgaccctcagtgtccagctccagccctatgatccgtcgtgctgtttgggctgtccgcttcccactgcaccgggcagggctgtaggcatcaatctcttccaggaggatgggctcaggtcccccggatcgcccacctggggtcagcaccttcagcactgtcccatcattggagccaaggaacatgactgtgatgttactgtggggaccagccatgccatccacagctacttgggtcagtagggccctgctagtgagagtgagtagaggctgatgggtgacaggtggtacagcggggtccagcagcgggtgagccttgatgaaggtcaggacatcatcagggaggtctcgggaagaggagaacaaggcagctccccctactcctgcacaggatcctggcctgggtgagggaactctgtcctcagacacaggagtccaggccccatccagactcctctgctccttgaacttgccctcaaacccacgctcaatctcatccaggtagaaggcgcagacggcagagccagggatgctattggtctgggtggtgaagaccccaaagagagcagagcggccatgcaggttcacaggcccagtcaaggcctgtaaaacatcaaaatagaaagtagagtccccagggacagagcagttgagccgaagcttcaggaaggatgtccagtggcggtccaaggcccgaggcgagccgcccatgtcacgtttacatactcgggctacgcgggagaactgcaccctccccagccgagcatcctccacagagacctcgcggaagaagaagtagacatggtctccatgctccaaggcctggacaaagtgtggctttggcggagcggagtgggggctggggcccaaggcttctgtaaactacagcatcactggcctggaaatccgcagctgtggctgagtacaggctgccctctgcaaagatggccacgt

SEQ ID NO: 9492 - RNA, 616 nt, Homo sapiens
  source 1..616: mol_type = other RNA
agggggtagaaagtggctgaagaggccccagaaggggttcttccagcattcatttgtgcattggattcccccaatgactgaagttcatattgaatagcctgcccattttggtccactagatggaattgctctgcagaaagagtctgtgtctgagtcaggggccctggtatattctgtgatatgagtgaattatttgcttcacgagtagtgatgggcaaaactgtaggagaatcattttgtccaaaggaagaatccctggagtccatacagattagatgctcaaatacttgagcactggtttttgactcttcaccgtcattatggttgactcttaatgaatcattagattgttccatgctgacatcatattcaattccattttcttctattatttaatagcttcagatagtggctcaggtttaaattccaggcctcaagcattctactacccccagaaatgtcctttcttgtccactgaagttcttccttttgggggcactaaatcatgatagctgtagcttcatttatgtgaaagctttaattgggtcttcacagcagcattttctctcgtcttggctccgaggccccgccatggagaccagcataatgcgcaggc

SEQ ID NO: 9493 - RNA, 622 nt, Homo sapiens
  source 1..622: mol_type = other RNA
agggggtagaaagtggctgaagaggccccagaaggggttcttccagcattccggtcactgactttttgggcaatgggaaggatgtttgaggatgaagaatgtaattgctggtattgtctgctagagtatccactcttacagttggtaagtttctgttactgggtttctcttcagggacatcccgaggactattcacatccacaagttgcccctgaggtataatcacttgtgccattcctgtctgggtaggtggaattacacgaagtacctgtccattttctgttgggctggcaacgatcatcatttgtgcattggattcccccaatgactgaagttcatattgaatagcctgcccattttggtccactagatggaattgctctgcagaaagagtctgtgtctgagtcaggggccctggtatattctgtgatatgagtgaattatttgcttcacgagtagtgatgggcaaaactgtaggagaatcattttgtccaaaggaagaatccctggagtccatacagattagatgctcaaatacttgagcactggtttttgactcttcaccgtcattatggttgactcttaatgaatcattagattgttccatgctgacatcatattc

SEQ ID NO: 9494 - RNA, 1764 nt, Homo sapiens
  source 1..1764: mol_type = other RNA
agggggtagaaagtggctgaagaggccccagaaggggttcttccagcattccggtcactgactttttgggcaatgggaaggatgtttgaggatgaagaatgtaattgctggtattgtctgctagagtatccactcttacagttggtaagtttctgttactgggtttctcttcagggacatcccgaggactattcacatccacaagttgcccctgaggtataatcacttgtgccattcctgtctgggtaggtggaattacacgaagtacctgtccattttctgttgggctggcaacgatcatcatttgtgcattggattcccccaatgactgaagttcatattgaatagcctgcccattttggtccactagatggaattgctctgcagaaagagtctgtgtctgagtcaggggccctggtatattctgtgatatgagtgaattatttgcttcacgagtagtgatgggcaaaactgtaggagaatcattttgtccaaaggaagaatccctggagtccatacagattagatgctcaaatacttgagcactggtttttgactcttcaccgtcattatggttgactcttaatgaatcattagattgttccatgctgacatcatattcaattccattttcttctattatttaatagctcacaccagatagcaaatcaacttgaaatggatcacagactatcaaatgataaaacttctagaagaaaacacaggagaaaatctttgtacccttggacttggcaaagatatattaaaccttcagatagtggctcaggtttaaattccaggcctcaagcattctactacccccagaaatgtcctttcttgtccactgaagttcttccttttgggggcactaaatcatgatagctgtagcttcatttatgtgaaagctttaattgggtcttcacagcagcattttctcggtctgcccataaattttgcaatccagttctgcctgattctaaactgcttgtctcttgaagcgaatgccttaaaaagtgacattgggatcaggatagttatctccatccatcctccctcagaaaaacaactatattagagtaattcttgggaccattgagaacaatacacaggcctttgggtaacttcaagacaaaaaaggcaaaaagtcggggagaaggtgtgggaggatgattttccccttctaaacgtaaggtataaaagggctcagaaagcggaaaaagaaccctaaaaagcaaggtgcgggacggcgtgagggaccacacattgggcgctccgcccaaggggtccggctccttctccgcggcgatggcgcgtccttgggctcagcaaccctcctgaagacacctaacctcctccttctccagcctgcccctctggggcctgcgagccccgtcccgggccgggggtcggaagccgtgccatgtgggaccccgaaaaggcccccaagcttggcgcggaaggcgccgccagtgaccggctgcggctgggggcggaggccggcagttgctcggagctccggcgggtcaggaggtgacgggaggaggaggaggcaggaggaagacggggggttgggaggtagcgtccggtaggtctgcgcagacagcgctgccagacctctgactcccccagtcctgccgccgccgatagccccacaaggcgacatgggaagtccgccggagcagaggggagaaaattcaaaacgagtctactcaacctcgtcttggctccgaggccccgccatggagaccagcataatgcgcaggc

SEQ ID NO: 9495 - RNA, 982 nt, Homo sapiens
  source 1..982: mol_type = other RNA
agggggtagaaagtggctgaagaggccccagaaggggttcttccagcattccggtcactgactttttgggcaatgggaaggatgtttgaggatgaagaatgtaattgctggtattgtctgctagagtatccactcttacagttggtaagtttctgttactgggtttctcttcagggacatcccgaggactattcacatccacaagttgcccctgaggtataatcacttgtgccattcctgtctgggtaggtggaattacacgaagtacctgtccattttctgttgggctggcaacgatcatcatttgtgcattggattcccccaatgactgaagttcatattgaatagcctgcccattttggtccactagatggaattgctctgcagaaagagtctgtgtctgagtcaggggccctggtatattctgtgatatgagtgaattatttgcttcacgagtagtgatgggcaaaactgtaggagaatcattttgtccaaaggaagaatccctggagtccatacagattagatgctcaaatacttgagcactggtttttgactcttcaccgtcattatggttgactcttaatgaatcattagattgttccatgctgacatcatattcaattccattttcttctattatttaatagctcacaccagatagcaaatcaacttgaaatggatcacagactatcaaatgataaaacttctagaagaaaacacaggagaaaatctttgtacccttggacttggcaaagatatattaaaccttcagatagtggctcaggtttaaattccaggcctcaagcattctactacccccagaaatgtcctttcttgtccactgaagttcttccttttgggggcactaaatcatgatagctgtagcttcatttatgtgaaagctttaattgggtcttcacagcagcattttctctcgtcttggctccgaggccccgccatggagaccagcataatgcgc

SEQ ID NO: 9496 - RNA, 926 nt, Homo sapiens
  source 1..926: mol_type = other RNA
agggggtagaaagtggctgaagaggccccagaaggggttcttccagcattccggtcactgactttttgggcaatgggaaggatgtttgaggatgaagaatgtaattgctggtattgtctgctagagtatccactcttacagttggtaagtttctgttactgggtttctcttcagggacatcccgaggactattcacatccacaagttgcccctgaggtataatcacttgtgccattcctgtctgggtaggtggaattacacgaagtacctgtccattttctgttgggctggcaacgatcatcatttgtgcattggattcccccaatgactgaagttcatattgaatagcctgcccattttggtccactagatggaattgctctgcagaaagagtctgtgtctgagtcaggggccctggtatattctgtgatatgagtgaattatttgcttcacgagtagtgatgggcaaaactgtaggagaatcattttgtccaaaggaagaatccctggagtccatacagattagatgctcaaatacttgagcactggtttttgactcttcaccgtcattatggttgactcttaatgaatcattagattgttccatgctgacatcatattcaattccattttcttctattatttaatagctcacaccagatagcaaatcaacttgaaatggatcacagactatcaaatgataaaacttcttcagatagtggctcaggtttaaattccaggcctcaagcattctactacccccagaaatgtcctttcttgtccactgaagttcttccttttgggggcactaaatcatgatagctgtagcttcatttatgtgaaagctttaattgggtcttcacagcagcattttctctcgtcttggctccgaggccccgccatggagaccagcataatgcgcaggc

SEQ ID NO: 9497 - RNA, 961 nt, Homo sapiens
  source 1..961: mol_type = other RNA
agggggtagaaagtggctgaagaggccccagaaggggttcttccagcattccggtcactgactttttgggcaatgggaaggatgtttgaggatgaagaatgtaattgctggtattgtctgctagagtatccactcttacagttggtaagtttctgttactgggtttctcttcagggacatcccgaggactattcacatccacaagttgcccctgaggtataatcacttgtgccattcctgtctgggtaggtggaattacacgaagtacctgtccattttctgttgggctggcaacgatcatcatttgtgcattggattcccccaatgactgaagttcatattgaatagcctgcccattttggtccactagatggaattgctctgcagaaagagtctgtgtctgagtcaggggccctggtatattctgtgatatgagtgaattatttgcttcacgagtagtgatgggcaaaactgtaggagaatcattttgtccaaaggaagaatccctggagtccatacagattagatgctcaaatacttgagcactggtttttgactcttcaccgtcattatggttgactcttaatgaatcattagattgttccatgctgacatcatattcaattccattttcttctattatttaatagctgcagtcccaggtaatcagatggctgaggtgggaggatcacttgatcctgggaggttaagactgcagtcagctgtgatcatagcactgcactccagccttcagatagtggctcaggtttaaattccaggcctcaagcattctactacccccagaaatgtcctttcttgtccactgaagttcttccttttgggggcactaaatcatgatagctgtagcttcatttatgtgaaagctttaattgggtcttcacagcagcattttctctcgtcttggctccgaggccccgccatggagaccagcataatgcgc

SEQ ID NO: 9498 - RNA, 930 nt, Homo sapiens
  source 1..930: mol_type = other RNA
agggggtagaaagtggctgaagaggccccagaaggggttcttccagcattccggtcactgactttttgggcaatgggaaggatgtttgaggatgaagaatgtaattgctggtattgtctgctagagtatccactcttacagttggtaagtttctgttactgggtttctcttcagggacatcccgaggactattcacatccacaagttgcccctgaggtataatcacttgtgccattcctgtctgggtaggtggaattacacgaagtacctgtccattttctgttgggctggcaacgatcatcatttgtgcattggattcccccaatgactgaagttcatattgaatagcctgcccattttggtccactagatggaattgctctgcagaaagagtctgtgtctgagtcaggggccctggtatattctgtgatatgagtgaattatttgcttcacgagtagtgatgggcaaaactgtaggagaatcattttgtccaaaggaagaatccctggagtccatacagattagatgctcaaatacttgagcactggtttttgactcttcaccgtcattatggttgactcttaatgaatcattagattgttccatgctgacatcatattcaattccattttcttctattatttaatagcttcagatagtggctcaggtttaaattccaggcctcaagcattctactacccccagaaatgtcctttcttgtccactgaagttcttccttttgggggcactaaatcatgatagctgtagcttcatttatgtgaaagctttaattgggtcttcacagcagcattttctcggtctgcccataaattttgcaatccagttctgcctgattctaaactgcttgtctcttgaagcgaatgcctcgtcttggctccgaggccccgccatggagaccagcataatgc

SEQ ID NO: 9499 - RNA, 1526 nt, Homo sapiens
  source 1..1526: mol_type = other RNA
agggggtagaaagtggctgaagaggccccagaaggggttcttccagcattccggtcactgactttttgggcaatgggaaggatgtttgaggatgaagaatgtaattgctggtattgtctgctagagtatccactcttacagttggtaagtttctgttactgggtttctcttcagggacatcccgaggactattcacatccacaagttgcccctgaggtataatcacttgtgccattcctgtctgggtaggtggaattacacgaagtacctgtccattttctgttgggctggcaacgatcatcatttgtgcattggattcccccaatgactgaagttcatattgaatagcctgcccattttggtccactagatggaattgctctgcagaaagagtctgtgtctgagtcaggggccctggtatattctgtgatatgagtgaattatttgcttcacgagtagtgatgggcaaaactgtaggagaatcattttgtccaaaggaagaatccctggagtccatacagattagatgctcaaatacttgagcactggtttttgactcttcaccgtcattatggttgactcttaatgaatcattagattgttccatgctgacatcatattcaattccattttcttctattatttaatagcttcagatagtggctcaggtttaaattccaggcctcaagcattctactacccccagaaatgtcctttcttgtccactgaagttcttccttttgggggcactaaatcatgatagctgtagcttcatttatgtgaaagctttaattgggtcttcacagcagcattttctcggtctgcccataaattttgcaatccagttctgcctgattctaaactgcttgtctcttgaagcgaatgccttaaaaagtgacattgggatcaggatagttatctccatccatcctccctcagaaaaacaactatattagagtaattcttgggaccattgagaacaatacacaggcctttgggtaacttcaagacaaaaaaggcaaaaagtcggggagaaggtgtgggaggatgattttccccttctaaacgtaaggtataaaagggctcagaaagcggaaaaagaaccctaaaaagcaaggtgcgggacggcgtgagggaccacacattgggcgctccgcccaaggggtccggctccttctccgcggcgatggcgcgtccttgggctcagcaaccctcctgaagacacctaacctcctccttctccagcctgcccctctggggcctgcgagccccgtcccgggccgggggtcggaagccgtgccatgtgggaccccgaaaaggcccccaagcttggcgcggaaggcgccgccagtgaccggctgcggctgggggcggaggccggcagttgctcggagctccggcgggtcaggaggtgacgggaggaggaggaggcaggaggaagacggggggttgggaggtagcgtccggtaggtctgcgcagacagcgctgccagacctctgactcccccagtcctgccgccgccgat

SEQ ID NO: 9500 - RNA, 863 nt, Homo sapiens
  source 1..863: mol_type = other RNA
agggggtagaaagtggctgaagaggccccagaaggggttcttccagcattccggtcactgactttttgggcaatgggaaggatgtttgaggatgaagaatgtaattgctggtattgtctgctagagtatccactcttacagttggtaagtttctgttactgggtttctcttcagggacatcccgaggactattcacatccacaagttgcccctgaggtataatcacttgtgccattcctgtctgggtaggtggaattacacgaagtacctgtccattttctgttgggctggcaacgatcatcatttgtgcattggattcccccaatgactgaagttcatattgaatagcctgcccattttggtccactagatggaattgctctgcagaaagagtctgtgtctgagtcaggggccctggtatattctgtgatatgagtgaattatttgcttcacgagtagtgatgggcaaaactgtaggagaatcattttgtccaaaggaagaatccctggagtccatacagattagatgctcaaatacttgagcactggtttttgactcttcaccgtcattatggttgactcttaatgaatcattagattgttccatgctgacatcatattcaattccattttcttctattatttaatagcttcagatagtggctcaggtttaaattccaggcctcaagcattctactacccccagaaatgtcctttcttgtccactgaagttcttccttttgggggcactaaatcatgatagctgtagcttcatttatgtgaaagctttaattgggtcttcacagcagcattttctctcgtcttggctccgaggccccgccatggagaccagcataatgcgc

SEQ ID NO: 9501 - RNA, 867 nt, Homo sapiens
  source 1..867: mol_type = other RNA
agggggtagaaagtggctgaagaggccccagaaggggttcttccagcattccggtcactgactttttgggcaatgggaaggatgtttgaggatgaagaatgtaattgctggtattgtctgctagagtatccactcttacagttggtaagtttctgttactgggtttctcttcagggacatcccgaggactattcacatccacaagttgcccctgaggtataatcacttgtgccattcctgtctgggtaggtggaattacacgaagtacctgtccattttctgttgggctggcaacgatcatcatttgtgcattggattcccccaatgactgaagttcatattgaatagcctgcccattttggtccactagatggaattgctctgcagaaagagtctgtgtctgagtcaggggccctggtatattctgtgatatgagtgaattatttgcttcacgagtagtgatgggcaaaactgtaggagaatcattttgtccaaaggaagaatccctggagtccatacagattagatgctcaaatacttgagcactggtttttgactcttcaccgtcattatggttgactcttaatgaatcattagattgttccatgctgacatcatattcaattccattttcttctattatttaatagcttcagatagtggctcaggtttaaattccaggcctcaagcattctactacccccagaaatgtcctttcttgtccactgaagttcttccttttgggggcactaaatcatgatagctgtagcttcatttatgtgaaagctttaattgggtcttcacagcagcattttctctcgtcttggctccgaggccccgccatggagaccagcataatgcgcaggc

SEQ ID NO: 9502 - RNA, 1657 nt, Homo sapiens
  source 1..1657: mol_type = other RNA
agggggtagaaagtggctgaagaggccccagaaggggttcttccagcattccggtcactgactttttgggcaatgggaaggatgtttgaggatgaagaatgtaattgctggtattgtctgctagagtatccactcttacagttggtaagtttctgttactgggtttctcttcagggacatcccgaggactattcacatccacaagttgcccctgaggtataatcacttgtgccattcctgtctgggtaggtggaattacacgaagtacctgtccattttctgttgggctggcaacgatcatcatttgtgcattggattcccccaatgactgaagttcatattgaatagcctgcccattttggtccactagatggaattgctctgcagaaagagtctgtgtctgagtcaggggccctggtatattctgtgatatgagtgaattatttgcttcacgagtagtgatgggcaaaactgtaggagaatcattttgtccaaaggaagaatccctggagtccatacagattagatgctcaaatacttgagcactggtttttgactcttcaccgtcattatggttgactcttaatgaatcattagattgttccatgctgacatcatattcaattccattttcttctattatttaatagcttcagatagtggctcaggtttaaattccaggcctcaagcattctactacccccagaaatgtcctttcttgtccactgaagttcttccttttgggggcactaaatcatgatagctgtagcttcatttatgtgaaagctttaattgggtcttcacagcagcattttctctgcacacataccggtctgcccataaattttgcaatccagttctgcctgattctaaactgcttgtctcttgaagcgaatgccttaaaaagtgacattgggatcaggatagttatctccatccatcctccctcagaaaaacaactatattagagtaattcttgggaccattgagaacaatacacaggcctttgggtaacttcaagacaaaaaaggcaaaaagtcggggagaaggtgtgggaggatgattttccccttctaaacgtaaggtataaaagggctcagaaagcggaaaaagaaccctaaaaagcaaggtgcgggacggcgtgagggaccacacattgggcgctccgcccaaggggtccggctccttctccgcggcgatggcgcgtccttgggctcagcaaccctcctgaagacacctaacctcctccttctccagcctgcccctctggggcctgcgagccccgtcccgggccgggggtcggaagccgtgccatgtgggaccccgaaaaggcccccaagcttggcgcggaaggcgccgccagtgaccggctgcggctgggggcggaggccggcagttgctcggagctccggcgggtcaggaggtgacgggaggaggaggaggcaggaggaagacggggggttgggaggtagcgtccggtaggtctgcgcagacagcgctgccagacctctgactcccccagtcctgccgccgccgatagccccacaaggcgacatgggaagtccgccggagcagaggggagaaaattcaaaacgagtctactcaacctcgtcttggctccgaggccccgccatggagaccagcataatgcgcaggc

SEQ ID NO: 9503 - RNA, 744 nt, Homo sapiens
  source 1..744: mol_type = other RNA
agggggtagaaagtggctgaagaggccccagaaggggttcttccagcattccggtcactgactttttgggcaatgggaaggatgtttgaggatgaagaatgtaattgctggtattgtctgctagagtatccactcttacagttggtaagtttctgttactgggtttctcttcagggacatcccgaggactattcacatccacaagttgcccctgaggtataatcacttgtgccattcctgtctgggtaggtggaattacacgaagtacctgtccattttctgttgggctggcaacgatcatcatttgtgcattggattcccccaatgactgaagttcatattgaatagcctgcccattttggtccactagatggaattgctctgcagaaagagtctgtgtctgagtcaggggccctggtatattctgtgatatgagtgaattatttgcttcacgagtagtgatgggcaaaactgtaggagaatcattttgtccaaaggaagaatccctggagtccatacagattagatgcttcagatagtggctcaggtttaaattccaggcctcaagcattctactacccccagaaatgtcctttcttgtccactgaagttcttccttttgggggcactaaatcatgatagctgtagcttcatttatgtgaaagctttaattgggtcttcacagcagcattttctctcgtcttggctccgaggccccgccatggagaccagcataatgcgcag

SEQ ID NO: 9504 - RNA, 746 nt, Homo sapiens
  source 1..746: mol_type = other RNA
agggggtagaaagtggctgaagaggccccagaaggggttcttccagcattccggtcactgactttttgggcaatgggaaggatgtttgaggatgaagaatgtaattgctggtattgtctgctagagtatccactcttacagttggtaagtttctgttactgggtttctcttcagggacatcccgaggactattcacatccacaagttgcccctgaggtataatcacttgtgccattcctgtctgggtaggtggaattacacgaagtacctgtccattttctgttgggctggcaacgatcatcatttgtgcattggattcccccaatgactgaagttcatattgaatagcctgcccattttggtccactagatggaattgctctgcagaaagagtctgtgtctgagtcaggggccctggtatattctgtgatatgagtgaattatttgcttcacgagtagtgatgggcaaaactgtaggagaatcattttgtccaaaggaagaatccctggagtccatacagattagatgcttcagatagtggctcaggtttaaattccaggcctcaagcattctactacccccagaaatgtcctttcttgtccactgaagttcttccttttgggggcactaaatcatgatagctgtagcttcatttatgtgaaagctttaattgggtcttcacagcagcattttctctcgtcttggctccgaggccccgccatggagaccagcataatgcgcaggc

SEQ ID NO: 9505 - RNA, 551 nt, Homo sapiens
  source 1..551: mol_type = other RNA
agggggtagaaagtggctgaagaggccccagaaggggttcttccagcattccggtcactgactttttgggcaatgggaaggatgtttgaggatgaagaatgtaattgctggtattgtctgctagagtatccactcttacagttggtaagtttctgttactgggtttctcttcagggacatcccgaggactattcacatccacaagttgcccctgaggtataatcacttgtgccattcctgtctgggtaggtggaattacacgaagtacctgtccattttctgttgggctggcaacgatcatcatttgtgcattggattcccccaatgactgaagttcatattgaatagcctgcccattttggtccactagatggaattgctctgcagaaagagtctgtgtctgagtcaggggccctggtatattctgtgatatgagtgaattatttgcttcacgagtagtgatgggcaaaactgtaggagaatcattttgtccaaaggaagaatccctggagtccatacagattagatgtatcttaattttaccaaaattg

SEQ ID NO: 9506 - RNA, 639 nt, Homo sapiens
  source 1..639: mol_type = other RNA
agggggtagaaagtggctgaagaggccccagaaggggttcttccagcattccggtcactgactttttgggcaatgggaaggatgtttgaggatgaagaatgtaattgctggtattgtctgctagagtatccactcttacagttggtaagtttctgttactgggtttctcttcagggacatcccgaggactattcacatccacaagttgcccctgaggtataatcacttgtgccattcctgtctgggtaggtggaattacacgaagtacctgtccattttctgttgggctggcaacgatcatctcaaatacttgagcactggtttttgactcttcaccgtcattatggttgactcttaatgaatcattagattgttccatgctgacatcatattcaattccattttcttctattatttaatagcttcagatagtggctcaggtttaaattccaggcctcaagcattctactacccccagaaatgtcctttcttgtccactgaagttcttccttttgggggcactaaatcatgatagctgtagcttcatttatgtgaaagctttaattgggtcttcacagcagcattttctctcgtcttggctccgaggccccgccatggagaccagcataatgcgcaggc

SEQ ID NO: 9507 - RNA, 720 nt, Homo sapiens
  source 1..720: mol_type = other RNA
agggggtagaaagtggctgaagaggccccagaaggggttcttccagcattccggtcactgactttttgggcaatgggaaggatgtttgaggatgaagaatgtaattgctggtattgtctgctagagtatccactcttacagttggtaagtttctgttactgggtttctcttcagggacatcccgaggactattcacatccacaagttgcccctgaggtataatcacttgtgccattcctgtctgggtaggtggaattacacgaagtacctgtccattttctgttgggctggcaacgatcatctcaaatacttgagcactggtttttgactcttcaccgtcattatggttgactcttaatgaatcattagattgttccatgctgacatcatattcaattccattttcttctattatttaatagcttcagatagtggctcaggtttaaattccaggcctcaagcattctactacccccagaaatgtcctttcttgtccactgaagttcttccttttgggggcactaaatcatgatagctgtagcttcatttatgtgaaagctttaattgggtcttcacagcagcattttctctgcacacataccggtctgcccataaattttgcaatccagttctgcctgattctaaactgcttgtctcttgaagcgaatgcctcgtcttggctccgaggccccgccatggagaccagcataatgcgcaggc

SEQ ID NO: 9508 - RNA, 637 nt, Homo sapiens
  source 1..637: mol_type = other RNA
agggggtagaaagtggctgaagaggccccagaaggggttcttccagcattccggtcactgactttttgggcaatgggaaggatgtttgaggatgaagaatgtaattgctggtattgtctgctagagtatccactcttacagttggtaagtttctgttactgggtttctcttcagggacatcccgaggactattcacatccacaagttgcccctgaggtataatcacttgtgccattcctgtctgggtaggtggaattacacgaagtacctgtccattttctgttgggctggcaacgatcatctcacaccagatagcaaatcaacttgaaatggatcacagactatcaaatgataaaacttctagaagaaaacacaggagaaaatctttgtacccttggacttggcaaagatatattaaaccttcagatagtggctcaggtttaaattccaggcctcaagcattctactacccccagaaatgtcctttcttgtccactgaagttcttccttttgggggcactaaatcatgatagctgtagcttcatttatgtgaaagctttaattgggtcttcacagcagcattttctctcgtcttggctccgaggccccgccatggagaccagcataatgcgcaggc

SEQ ID NO: 9509 - RNA, 323 nt, Homo sapiens
  source 1..323: mol_type = other RNA
agggggtagaaagtggctgaagaggccccagaaggggttcttccagcattccggtcactgactttttgggcaatgggaaggatgtttgaggatgaagaatgtaattgctggtattgtctgctagagtatccactcttacagttggtaagtttctgttactgggtttctcttcagggacatcccgaggactattcacatccacaagttgcccctgaggtataatcacttgtgccattcctgtctgggtaggtggaattacacgaagtacctgtccattttctgttgggctggcaacgatcatctgtaatcctagcactttggga

SEQ ID NO: 9510 - RNA, 414 nt, Homo sapiens
  source 1..414: mol_type = other RNA
agggggtagaaagtggctgaagaggccccagaaggggttcttccagcattccggtcactgactttttgggcaatgggaaggatgtttgaggatgaagaatgtaattgctggtattgtctgctagagtatccactcttacagttggtaagtttctgttactgggtttctcttcagggacatcccgaggactattcacatccacaagttgcccctgaggtataatcacttgtgccattcctgtctgggtaggtggaattacacgaagtacctgtccattttctgttgggctggcaacgatcatctgtaatcctagcactttgggaggccaaggaaggcagatcacgaggtcaggagttcgagaccagcctgatcaacatggtgaaaccctgtctccactaaaaatacaaaaattag

SEQ ID NO: 9511 - RNA, 518 nt, Homo sapiens
  source 1..518: mol_type = other RNA
agggggtagaaagtggctgaagaggccccagaaggggttcttccagcattccggtcactgactttttgggcaatgggaaggatgtttgaggatgaagaatgtaattgctggtattgtctgctagagtatccactcttacagttggtaagtttctgttactgggtttctcttcagggacatcccgaggactattcacatccacaagttgcccctgaggtataatcacttgtgccattcctgtctgggtaggtggaattacacgaagtacctgtccattttctgttgggctggcaacgatcatcttcagatagtggctcaggtttaaattccaggcctcaagcattctactacccccagaaatgtcctttcttgtccactgaagttcttccttttgggggcactaaatcatgatagctgtagcttcatttatgtgaaagctttaattgggtcttcacagcagcattttctctcgtcttggctccgaggccccgccatggagaccagcataatgcgcaggc

SEQ ID NO: 9512 - RNA, 626 nt, Homo sapiens
  source 1..626: mol_type = other RNA
agggggtagaaagtggctgaagaggccccagaaggggttcttccagcattccggtcactgactttttgggcaatgggaaggatgtttgaggatgaagaatgtaattgctggtattgtctgctagagtatccactcttacagttggtaagtttctgttactgggtttctcttcagggacatcccgaggactattcacatccacaagttgcccctgaggtataatcacttgtgccattcctgtctgggtaggtggaattacacgaagtacctgtccattttctgttgggctggcaacgatcatcttcagatagtggctcaggtttaaattccaggcctcaagcattctactacccccagaaatgtcctttcttgtccactgaagttcttccttttgggggcactaaatcatgatagctgtagcttcatttatgtgaaagctttaattgggtcttcacagcagcattttctctgcacacataccggtctgcccataaattttgcaatccagttctgcctgattctaaactgcttgtctcttgaagcgaatgcctcgtcttggctccgaggccccgccatggagaccagcataatgcgcaggcgcgccccaccgggagcgcgcagagcag

SEQ ID NO: 9513 - RNA, 529 nt, Homo sapiens
  source 1..529: mol_type = other RNA
agggggtagaaagtggctgaagaggccccagaaggggttcttccagcattccggtcactgactttttgggcaatgggaaggatgtttgaggatgaagaatgtaattgctggtattgtctgctagagtatccactcttacagttggtaagtttctgttactgggtttctcttcagggacatcccgaggactattcacatccacaagttgcccctgaggtataatcacttgtgccattcctgtctgggtaggtggaattacacgaagtacctgtccattttctgttgggctggcaacgatcattttgtatagaaagtttaatccaattacaaagagtgttaattaacttttttttggactcaaataaacaattttgctcggaaaggtaccctaggtaaaatgacaacccttttacacattcagactccttgatcttccatttgtgcattggattcccccaatgactgaagttcatattgaatagcctgcccattttggtccactagatggaattgctctgcagaaagagtc

SEQ ID NO: 9514 - RNA, 516 nt, Homo sapiens
  source 1..516: mol_type = other RNA
agggtggggctggaggtggggctggacactcggggtgaccctggtggagcccctcaagtccctgggaagttgacggccaggcaggattcacactccaacctggggcttgaccacggggtctccaagaagaggagcccctgcacccctctcctggctccgcagtgcgttgtcctcgaggcttttccgtgtgtttccaccccgggaggctccttctcccttgtccactacattctttggtgcattctcagtggtgatgggcaccagctcatggttggatggaggaacgcagggggcagccacctttcctgcagaggagccactaagtcaggtgggtgtctgggccaagggactcccaggacaggggcggtggccagtggcggaggcagcagctgtggctggcaagaagctggtttcccccagaagaaggcagcgagtgagcctgtgtccaggcagggagcggggtgcaaggagcagagctggtcccagggccactgctgggagcaactgagcagaggg

SEQ ID NO: 9515 - RNA, 186 nt, Homo sapiens
  source 1..186: mol_type = other RNA
agggtggggctggaggtggggctggacactcggggtgaccctggtggagccgttgtcctcgaggcttttccgtgtgtttccaccccgggaggctccttctcccttgtccactacattctttggtgcattctcagtggtgatgggcaccagctcatggttggatggaggaacgcagggggcagccac

SEQ ID NO: 9516 - RNA, 378 nt, Homo sapiens
  source 1..378: mol_type = other RNA
agggtggggctggaggtggggctggacactcggggtgaccctggtggagccgttgtcctcgaggcttttccgtgtgtttccaccccgggaggctccttctcccttgtccactacattctttggtgcattctcagtggtgatgggcaccagctcatggttggatggaggaacgcagggggcagccacctgcatgccactgggcctctgcacatgccttcccctgtgcctgaagaagtctttgccccttttcctccccgcaaaactccttgccaaacttcaaaatccatctcaaatggtacctcttctccaaagcttcctccgctctgccagctcacatgagctgcctcctgcttgacattcccactgcgttttgcagca

SEQ ID NO: 9517 - RNA, 339 nt, Homo sapiens
  source 1..339: mol_type = other RNA
agggtggggctggaggtggggctggacactcggggtgaccctggtggagccgttgtcctcgaggcttttccgtgtgtttccaccccgggaggctccttctcccttgtccactacattctttggtgcattctcagtggtgatgggcaccagctcatggttggatggaggaacgcagggggcagccaccttggcctggcatttccgatgacaggagaagctgcagactttgcaggtgcagccttcctgggtgatgacctggcggcagatcccacagggcttcaccttcttgaaggtcttcaccttgaagcggtgtgtcttgggggcctccagatcctctgg

SEQ ID NO: 9518 - RNA, 495 nt, Homo sapiens
  source 1..495: mol_type = other RNA
agggtggggctggaggtggggctggacactcggggtgaccctggtggagccgttgtcctcgaggcttttccgtgtgtttccaccccgggaggctccttctcccttgtccactacattctttggtgcattctcagtggtgatgggcaccagctcatggttggatggaggaacgcagggggcagccaccttggcctggcatttccgatgacaggagaagctgcagactttgcaggtgcagccttcctgggtgatgacctggcggcagatcccacagggcttcaccttcttgaaggtcttcaccttgaagcggtgtgtcttgggggcctccagatcctctggccagagcatgcaggacagacagatccacgtcatctttgctgggtcccgtcactgaggcacgcccagggcctgtgaagagcccctgaagctagagtccccgcggcgctggcagaagggctctctgagtccgcggctgctccggctccgccagcatct

SEQ ID NO: 9519 - RNA, 392 nt, Homo sapiens
  source 1..392: mol_type = other RNA
agggtggggctggaggtggggctggacactcggggtgaccctggtggagccgttgtcctcgaggcttttccgtgtgtttccaccccgggaggctccttctcccttgtccactacattctttggtgcattctcagtggtgatgggcaccagctcatggttggatggaggaacgcagggggcagccacctttcctgcagaggagccactaagtcaggtgggtgtctgggccaagggactcccaggacaggggcggtggccagtggcggaggcagcagctgtggctggcaagaagctggtttcccccagaagaaggcagcgagtgagcctgtgtccaggcagggagcggggtgcaaggagcagagctggtcccagggccactgctgggagcaact

SEQ ID NO: 9520 - RNA, 402 nt, Homo sapiens
  source 1..402: mol_type = other RNA
agggtggggctggaggtggggctggacactcggggtgaccctggtggagccgttgtcctcgaggcttttccgtgtgtttccaccccgggaggctccttctcccttgtccactacattctttggtgcattctcagtggtgatgggcaccagctcatggttggatggaggaacgcagggggcagccacctttcctgcagaggagccactaagtcaggtgggtgtctgggccaagggactcccaggacaggggcggtggccagtggcggaggcagcagctgtggctggcaagaagctggtttcccccagaagaaggcagcgagtgagcctgtgtccaggcagggagcggggtgcaaggagcagagctggtcccagggccactgctgggagcaactgagcagaggg

SEQ ID NO: 9521 - RNA, 3106 nt, Homo sapiens
  source 1..3106: mol_type = other RNA
agggtggggctggaggtggggcttggtgggaggtgtttgaatcatgagggtggatccctcatggctgggtgctgtcttccggatagtgagttcttgtgagatctggtaatttaaaattatgtggcgcctcccagccacccttccttgttcttgtttctgttctcaccatgcaatgtgcctgcttccctttgccttccgccacgattggaagcttcctgaggcctccccagaagcacatgctactatgcttcctgtacagtctgcagaactgtgggccaattataccccttttcttataaatcacctagtctcaggtatttctttatagccatgcaagaacagcctaatacactgacagtttatggtctctaaaagatcacgcatatatggaaatattgatactttagtcaatttagtttacctttacaaaccattttaataaagtaaaaagggagtattcttggagcaaggaggcctcctgaccgtttgtcttgcttacagagcctccttagttcattattattttaagagaatcatttgaatgaatataatgatatagaaaagcctactgtcctttgcctatttcttttcctttcagactagagaactggatggaaagagtctttattctttcctttcatcttcaacttttgaataagtcatggtggatcatctaggcctcctgaaccccaatcttcaattgatgttagtcaggttttcagaattccctagggtatgtggtcttgaaaggcactggctcttcagtaagaggactaacaggaagtgacgtggtactgcttgctggactcatgtctgcactctcttgaagaactctcttcatctttaataataacgtcttgactgccgtgcagtcctgtaacatcagtctgaatggcagagaatctatgcctccgttttcttccacaccttgtagaggccaatccgcagatggactgttgggcattcggctgatgtgggaacacctggcttcttgatcaacgtcctttgttaatttcagggaaagattctgtttggaaggctcaggaaattctggttcttctcttttcttcatttctatcattggttccataggagtaagaactactgcggcacatgagacgacagagtgatatgagtcctcccggcaaacagaagggtgaagactctgttcctctaaaaattcaagatcaagcattagatcatcttcatccagttcacaagatcccaaattattcaaaacatccaaactgttcatttttgaagatgaagaacctgctctttgctttcttaaactattaacttcttctatatttccatctttcggtttcaaaatcattctgctactccctgcagtgccttctgacgaggatcgcagtctcctctctataaatcttccttcacgaaatggactgagactactggcaagaactttggcaggatttgcttcatatccatgtgatgttttgttaaaaatatgatgatcaccagaagtaggtattatctttgaatctgaaataggatggatcccttttacatgttccgctattgctttatgttgctcataaaatccaagtttccttggggagtttgtccccagcattgtttcaccattttgtaaccctatattttcttctctttcactatctgctggtaggttactctctgagtggctcacacttgtagcaggtagttcagcaatttgtaataacacttccttctgattagcagcagaggtttccggtaatgaattagattcagtgctacattgaccctctaacctatatttcccaggagacataattgcacagggaacagttcccgtaagttctgttgttgtctttgtaacagcagcagaattgagggacatctgagaggtagaatcattgtggccaaagttgtcacagtgggatgccatgcttccacttttagaaaatgcatccatttcagacacagaatcttcagtcaaggctaaaaattctgaaggtgtctgagctgtggtaagatcagcagaaagcaaaggagattgtaaagagcttcctgcccgttctgttacatccacagaacaggatggcgaagctcttactaatacaggttctctctcttggtactgtgtaacttccaatgagaattcagactgttgtaccaatgaaatggattggctctgtagaactggcttagaaaatttatagtgagatgaaaaagatttagggagtagcttccttgttgactgcttaacagaacgacgagtttggtcttctgtgaaaccagaatcatccccttcacttttgccagaacttagacaatttataaagacattcttgttagttgagtgctctttttccctttcaaaatcctctgtcaaagatcttgttatcttcttatttcgtgaactactaaaaccaacagaatgtcttcccctggtcttaatatgttcttccaaactcagtttctgcatattgctgtgaccaggttgagcaccatttgaaatactaaggttctggttggtaggctcttgcttaggctcactccccttcttatggtggaagctaatggaaggagtacggaatatgctcctccgtttacctgtgctacctgagcttgagttagtgctggaaggagaggaactgtggacaccaactgtattactggaagaaggtgaagaaggaagagaatcatgtcttctgttaatacttcttctgaatattggcaaccgggagaccagggtagatcgtcttgatcctgagtcccccattgggaatcaaaggcttgcactgtgaaagccaactttgcagcctccaattgtcttctatcccaggcttcatgggcttaagcttgagtcctaaggcaaaggatctacaggtaatgagcaagtgaaatctaaaagcagctgcttgtctatggaatcaccctgggacatggagagcccaaggcatcagcagaattggcactggcagcagcagggcttgcagtgttggcagcagcactaatgacagcagcggtgcagttagtgataacaacatatttggcagcagcaagagttcatttaactccttatacattagctccctgcacctcgagcatacacagccccggtctcgatggtaac

SEQ ID NO: 9522 - RNA, 1810 nt, Homo sapiens
  source 1..1810: mol_type = other RNA
agggtgtgtgtgtttttttttttttttgtttaaatttctgaatccaacagttggtcacagaggtcaagtattatcaaggctcctttgtcagttctcaatcgtgtctgactcatccatccttcaagtacatgcaaggctcaatagttttccagaggcagatgcctggggccatttaagatacagatgaaataggattatgaggtgaacccatttgagtaagaactttatccagccactggagggggccgtgcagatgtatctcaatccagcagggggtgctagtaacatcctggcggtggtattctgctccccagcccttcacaaagctcatacgtatagtacacatttttgtaagctcatagactgtctcaaatccatggttcacagactgtgccaataactgagcaaattcttggttgttaaaaattttcagactacacccactagggatcttgcaaacagtagtaggatgaaatccatgatggtagttgcagttccgactttgcacaaagatgctactgtcactaaggcattcggcatacacctcccctccaacataataaagatgaactccttttccaatatgccgcctggtgttttcaatagtggaattccggttaacattggagagcagcccaaggcagaaacggttcttattgttggaaggatcagtgaaaccatccaccaacacacttgtggaggaggcatggaacgcttcacccacacgattgttgagctcatagtagacaatagagcaccagtgttttggttcctcataagcaaccgcctgaacatctcctctgttgatttctgagggcaggggaggcgccatcatgtttgtgtccatcggctgagagccatcctgggtcatggggtcttcaggaggcaggtaagcaggtgggggcgtatcagctggcatctggaaagggcttcctgggtctgagctggtgggagagtgagggtaggtgctgctgctgctcccaggagagtttgggtaactgctattgggagagtgaggaaacgggtggctgttgggttgctggaaagaatctggaaaagtggcgttgagtggcatgtgaggctcattttgtcctaagttacggaactgagctaagaggctgtgctgaggattatattcgctgtgtcttggaaccagcacaggaggaagtacagggctttctactctcttatagtggtagggattgatgcagacctccttctgcttggaaccaaaaggaaactcacagcattccagtggttttagttcatggtggctctgaagatcgggccagcgccacacacggcagtaaatgacatgaggcagtcccttccggtgggagacttgcagcctgccatccagagagcggggaatggtgacacagttactcggttgccctgggcagctcaaggccttttccagttcctccatggcacctttctttttcttcagttttttcaccaaagcatcaacagctttctctgcccatttttcttcttcatcgccctgtttccacccaagaagtctcttcacagctggacttgtaaaggaaaataaacttgtcacattcataatgacagcactagttatactccttggatatggtgaaataaagctgtctccaaatgcaaaaggacagcagaagagatttgtttatttacagagaagtctctttaacttcttagtttgaagtccagaagagtagaaattaccattcctagtgtttaaaaaagtaacccagtcagcacaaagacagggagcagagtaaaggaacagttgttcaaccgcgaactcacgaatacacatgcagtg

SEQ ID NO: 9523 - RNA, 1841 nt, Homo sapiens
  source 1..1841: mol_type = other RNA
agggtgtgtgtgtttttttttttttttgtttaaatttctgaatccaacagttggtcacagaggtcaagtattatcaaggctcctttgtcagttctcaatcgtgtctgactcatccatccttcaagtacatgcaaggctcaatagttttccagaggcagatgcctggggccatttaagatacagatgaaataggattatgaggtgaacccatttgagtaagaactttatccagccactggagggggccgtgcagatgtatctcaatccagcagggggtgctagtaacatcctggcggtggtattctgctccccagcccttcacaaagctcatacgtatagtacacatttttgtaagctcatagactgtctcaaatccatggttcacagactgtgccaataactgagcaaattcttggttgttaaaaattttcagactacacccactagggatcttgcaaacagtagtaggatgaaatccatgatggtagttgcagttccgactttgcacaaagatgctactgtcactaaggcattcggcatacacctcccctccaacataataaagatgaactccttttccaatatgccgcctggtgttttcaatagtggaattccggttaacattggagagcagcccaaggcagaaacggttcttattgttggaaggatcagtgaaaccatccaccaacacacttgtggaggaggcatggaacgcttcacccacacgattgttgagctcatagtagacaatagagcaccagtgttttggttcctcataagcaaccgcctgaacatctcctctgttgatttctgagggcaggggaggcgccatcatgtttgtgtccatcggctgagagccatcctgggtcatggggtcttcaggaggcaggtaagcaggtgggggcgtatcagctggcatctggaaagggcttcctgggtctgagctggtgggagagtgagggtaggtgctgctgctgctcccaggagagtttgggtaactgctattgggagagtgaggaaacgggtggctgttgggttgctggaaagaatctggaaaagtggcgttgagtggcatgtgaggctcattttgtcctaagttacggaactgagctaagaggctgtgctgaggattatattcgctgtgtcttggaaccagcacaggaggaagtacagggctttctactctcttatagtggtagggattgatgcagacctccttctgcttggaaccaaaaggaaactcacagcattccagtggttttagttcatggtggctctgaagatcgggccagcgccacacacggcagtaaatgacatgaggcagtcccttccggtgggagacttgcagcctgccatccagagagcggggaatggtgacacagttactcggttgccctgggcagctcaaggccttttccagttcctccatggcacctttctttttcttcagttttttcaccaaagcatcaacagctttctctgcccatttttcttcttcatcgccctgtttccacccaagaagtctcttcacagctggacttgtaaaggaaaataaacttgtcacattcataatgacagcactagttatactccttggatatggtgaaataaagctgtctccaaatgcaaaaggacagcagaagagatttgtttatttacagagaagtctctttaacttcttagtttgaagtccagaagagtagaaattaccattcctagtgtttaaaaaagtaacccagtcagcacccgcgcgccgccgccgctgccgcgcgaccagggatcctctccaaattcccggcccggccggcgtgagcgcagcgcggccggggccggaggacggc

SEQ ID NO: 9524 - RNA, 1849 nt, Homo sapiens
  source 1..1849: mol_type = other RNA
agggtgtgtgtgtttttttttttttttgtttaaatttctgaatccaacagttggtcacagaggtcaagtattatcaaggctcctttgtcagttctcaatcgtgtctgactcatccatccttcaagtacatgcaaggctcaatagttttccagaggcagatgcctggggccatttaagatacagatgaaataggattatgaggtgaacccatttgagtaagaactttatccagccactggagggggccgtgcagatgtatctcaatccagcagggggtgctagtaacatcctggcggtggtattctgctccccagcccttcacaaagctcatacgtatagtacacatttttgtaagctcatagactgtctcaaatccatggttcacagactgtgccaataactgagcaaattcttggttgttaaaaattttcagactacacccactagggatcttgcaaacagtagtaggatgaaatccatgatggtagttgcagttccgactttgcacaaagatgctactgtcactaaggcattcggcatacacctcccctccaacataataaagatgaactccttttccaatatgccgcctggtgttttcaatagtggaattccggttaacattggagagcagcccaaggcagaaacggttcttattgttggaaggatcagtgaaaccatccaccaacacacttgtggaggaggcatggaacgcttcacccacacgattgttgagctcatagtagacaatagagcaccagtgttttggttcctcataagcaaccgcctgaacatctcctctgttgatttctgagggcaggggaggcgccatcatgtttgtgtccatcggctgagagccatcctgggtcatggggtcttcaggaggcaggtaagcaggtgggggcgtatcagctggcatctggaaagggcttcctgggtctgagctggtgggagagtgagggtaggtgctgctgctgctcccaggagagtttgggtaactgctattgggagagtgaggaaacgggtggctgttgggttgctggaaagaatctggaaaagtggcgttgagtggcatgtgaggctcattttgtcctaagttacggaactgagctaagaggctgtgctgaggattatattcgctgtgtcttggaaccagcacaggaggaagtacagggctttctactctcttatagtggtagggattgatgcagacctccttctgcttggaaccaaaaggaaactcacagcattccagtggttttagttcatggtggctctgaagatcgggccagcgccacacacggcagtaaatgacatgaggcagtcccttccggtgggagacttgcagcctgccatccagagagcggggaatggtgacacagttactcggttgccctgggcagctcaaggccttttccagttcctccatggcacctttctttttcttcagttttttcaccaaagcatcaacagctttctctgcccatttttcttcttcatcgccctgtttccacccaagaagtctcttcacagctggacttgtaaaggaaaataaacttgtcacattcataatgacagcactagttatactccttggatatggtgaaataaagctgtctccaaatgcaaaaggacagcagaagagatttgtttatttacagagaagtctctttaacttcttagtttgaagtccagaagagtagaaattaccattcctagtgtttaaaaaagtaacccagtcagcacccgctcacccgcgcgccgccgccgctgccgcgcgaccagggatcctctccaaattcccggcccggccggcgtgagcgcagcgcggccggggccggaggacggc

SEQ ID NO: 9525 - RNA, 1932 nt, Homo sapiens
  source 1..1932: mol_type = other RNA
agggtgtgtgtgtttttttttttttttgtttaaatttctgaatccaacagttggtcacagaggtcaagtattatcaaggctcctttgtcagttctcaatcgtgtctgactcatccatccttcaagtacatgcaaggctcaatagttttccagaggcagatgcctggggccatttaagatacagatgaaataggattatgaggtgaacccatttgagtaagaactttatccagccactggagggggccgtgcagatgtatctcaatccagcagggggtgctagtaacatcctggcggtggtattctgctccccagcccttcacaaagctcatacgtatagtacacatttttgtaagctcatagactgtctcaaatccatggttcacagactgtgccaataactgagcaaattcttggttgttaaaaattttcagactacacccactagggatcttgcaaacagtagtaggatgaaatccatgatggtagttgcagttccgactttgcacaaagatgctactgtcactaaggcattcggcatacacctcccctccaacataataaagatgaactccttttccaatatgccgcctggtgttttcaatagtggaattccggttaacattggagagcagcccaaggcagaaacggttcttattgttggaaggatcagtgaaaccatccaccaacacacttgtggaggaggcatggaacgcttcacccacacgattgttgagctcatagtagacaatagagcaccagtgttttggttcctcataagcaaccgcctgaacatctcctctgttgatttctgagggcaggggaggcgccatcatgtttgtgtccatcggctgagagccatcctgggtcatggggtcttcaggaggcaggtaagcaggtgggggcgtatcagctggcatctggaaagggcttcctgggtctgagctggtgggagagtgagggtaggtgctgctgctgctcccaggagagtttgggtaactgctattgggagagtgaggaaacgggtggctgttgggttgctggaaagaatctggaaaagtggcgttgagtggcatgtgaggctcattttgtcctaagttacggaactgagctaagaggctgtgctgaggattatattcgctgtgtcttggaaccagcacaggaggaagtacagggctttctactctcttatagtggtagggattgatgcagacctccttctgcttggaaccaaaaggaaactcacagcattccagtggttttagttcatggtggctctgaagatcgggccagcgccacacacggcagtaaatgacatgaggcagtcccttccggtgggagacttgcagcctgccatccagagagcggggaatggtgacacagttactcggttgccctgggcagctcaaggccttttccagttcctccatggcacctttctttttcttcagttttttcaccaaagcatcaacagctttctctgcccatttttcttcttcatcgccctgtttccacccaagaagtctcttcacagctggacttgtaaaggaaaataaacttgtcacattcataatgacagcactagttatactccttggatatggtgaaataaagctgtctccaaatgcaaaaggacagcagaagagatttgtttatttacagagaagtctctttaacttcttagtttgaagtccagaagagtagaaattaccattcctagtgtttaaaaaagtaacccagtcagcaccgggttggcggcgcgcccgtccgtgtgggagcacgagtggccgggcgagcggggtctcgcggcccgggtccggacggccgggcgctgcgccactctccgctccccgagcctcggcccgggttgagccgctcggcctctcctttctccgcccgcccgcctgctttctcctggagcctggattgatct

SEQ ID NO: 9526 - RNA, 1841 nt, Homo sapiens
  source 1..1841: mol_type = other RNA
agggtgtgtgtgtttttttttttttttgtttaaatttctgaatccaacagttggtcacagaggtcaagtattatcaaggctcctttgtcagttctcaatcgtgtctgactcatccatccttcaagtacatgcaaggctcaatagttttccagaggcagatgcctggggccatttaagatacagatgaaataggattatgaggtgaacccatttgagtaagaactttatccagccactggagggggccgtgcagatgtatctcaatccagcagggggtgctagtaacatcctggcggtggtattctgctccccagcccttcacaaagctcatacgtatagtacacatttttgtaagctcatagactgtctcaaatccatggttcacagactgtgccaataactgagcaaattcttggttgttaaaaattttcagactacacccactagggatcttgcaaacagtagtaggatgaaatccatgatggtagttgcagttccgactttgcacaaagatgctactgtcactaaggcattcggcatacacctcccctccaacataataaagatgaactccttttccaatatgccgcctggtgttttcaatagtggaattccggttaacattggagagcagcccaaggcagaaacggttcttattgttggaaggatcagtgaaaccatccaccaacacacttgtggaggaggcatggaacgcttcacccacacgattgttgagctcatagtagacaatagagcaccagtgttttggttcctcataagcaaccgcctgaacatctcctctgttgatttctgagggcaggggaggcgccatcatgtttgtgtccatcggctgagagccatcctgggtcatggggtcttcaggaggcaggtaagcaggtgggggcgtatcagctggcatctggaaagggcttcctgggtctgagctggtgggagagtgagggtaggtgctgctgctgctcccaggagagtttgggtaactgctattgggagagtgaggaaacgggtggctgttgggttgctggaaagaatctggaaaagtggcgttgagtggcatgtgaggctcattttgtcctaagttacggaactgagctaagaggctgtgctgaggattatattcgctgtgtcttggaaccagcacaggaggaagtacagggctttctactctcttatagtggtagggattgatgcagacctccttctgcttggaaccaaaaggaaactcacagcattccagtggttttagttcatggtggctctgaagatcgggccagcgccacacacggcagtaaatgacatgaggcagtcccttccggtgggagacttgcagcctgccatccagagagcggggaatggtgacacagttactcggttgccctgggcagctcaaggccttttccagttcctccatggcacctttctttttcttcagttttttcaccaaagcatcaacagctttctctgcccatttttcttcttcatcgccctgtttccacccaagaagtctcttcacagctggacttgtaaaggaaaataaacttgtcacattcataatgacagcactagttatactccttggatatggtgaaataaagctgtctccaaatgcaaaaggacagcagaagagatttgtttatttacagagaagtctctttaacttcttagtttgaagtccagaagagtagaaattaccattcctagtgtttaaaaaagtaacccagtcagcacctttcgagacgcgcccttttatgtctatctttcgttgcccctcactcactctccaataatttgcaggccccagaagttgtacgtacccagaattg

SEQ ID NO: 9527 - RNA, 2120 nt, Homo sapiens
  source 1..2120: mol_type = other RNA
agggtgtgtgtgtttttttttttttttgtttaaatttctgaatccaacagttggtcacagaggtcaagtattatcaaggctcctttgtcagttctcaatcgtgtctgactcatccatccttcaagtacatgcaaggctcaatagttttccagaggcagatgcctggggccatttaagatacagatgaaataggattatgaggtgaacccatttgagtaagaactttatccagccactggagggggccgtgcagatgtatctcaatccagcagggggtgctagtaacatcctggcggtggtattctgctccccagcccttcacaaagctcatacgtatagtacacatttttgtaagctcatagactgtctcaaatccatggttcacagactgtgccaataactgagcaaattcttggttgttaaaaattttcagactacacccactagggatcttgcaaacagtagtaggatgaaatccatgatggtagttgcagttccgactttgcacaaagatgctactgtcactaaggcattcggcatacacctcccctccaacataataaagatgaactccttttccaatatgccgcctggtgttttcaatagtggaattccggttaacattggagagcagcccaaggcagaaacggttcttattgttggaaggatcagtgaaaccatccaccaacacacttgtggaggaggcatggaacgcttcacccacacgattgttgagctcatagtagacaatagagcaccagtgttttggttcctcataagcaaccgcctgaacatctcctctgttgatttctgagggcaggggaggcgccatcatgtttgtgtccatcggctgagagccatcctgggtcatggggtcttcaggaggcaggtaagcaggtgggggcgtatcagctggcatctggaaagggcttcctgggtctgagctggtgggagagtgagggtaggtgctgctgctgctcccaggagagtttgggtaactgctattgggagagtgaggaaacgggtggctgttgggttgctggaaagaatctggaaaagtggcgttgagtggcatgtgaggctcattttgtcctaagttacggaactgagctaagaggctgtgctgaggattatattcgctgtgtcttggaaccagcacaggaggaagtacagggctttctactctcttatagtggtagggattgatgcagacctccttctgcttggaaccaaaaggaaactcacagcattccagtggttttagttcatggtggctctgaagatcgggccagcgccacacacggcagtaaatgacatgaggcagtcccttccggtgggagacttgcagcctgccatccagagagcggggaatggtgacacagttactcggttgccctgggcagctcaaggccttttccagttcctccatggcacctttctttttcttcagttttttcaccaaagcatcaacagctttctctgcccatttttcttcttcatcgccctgtttccacccaagaagtctcttcacagctggacttgtaaaggaaaataaacttgtcacattcataatgacagcactagttatactccttggatatggtgaaataaagctgtctccaaatgcaaaaggacagcagaagagatttgtttatttacagagaagtctctttaacttcttagtttgaagtccagaagagtagaaattaccattcctagtgtttaaaaaagtaacccagtcagcacctttgaataaattagaggggatctcggtgcgaactttccttgacctcgaccccaaagaggcttgctggggccgagaagaaaacccgtgcgggatgtggaggggcccggggcgccggggtcccccgcccgcgagacccgctccaccaggcgccttggagagcagcgccagcggtcgtcctccagctcccgcaggggtcgccccgccggcgcgggggacacaatgggtccgcgggccacgcgaacgggcctcggcccggcggcagcacgggagagatgtgaggagcgcgcggaaggggagcgcggccggggagatcccagcgcggtcaggcccgggagccgaggctcgggggcccgggaactgggcttcccacagc

SEQ ID NO: 9528 - RNA, 2118 nt, Homo sapiens
  source 1..2118: mol_type = other RNA
agggtgtgtgtgtttttttttttttttgtttaaatttctgaatccaacagttggtcacagaggtcaagtattatcaaggctcctttgtcagttctcaatcgtgtctgactcatccatccttcaagtacatgcaaggctcaatagttttccagaggcagatgcctggggccatttaagatacagatgaaataggattatgaggtgaacccatttgagtaagaactttatccagccactggagggggccgtgcagatgtatctcaatccagcagggggtgctagtaacatcctggcggtggtattctgctccccagcccttcacaaagctcatacgtatagtacacatttttgtaagctcatagactgtctcaaatccatggttcacagactgtgccaataactgagcaaattcttggttgttaaaaattttcagactacacccactagggatcttgcaaacagtagtaggatgaaatccatgatggtagttgcagttccgactttgcacaaagatgctactgtcactaaggcattcggcatacacctcccctccaacataataaagatgaactccttttccaatatgccgcctggtgttttcaatagtggaattccggttaacattggagagcagcccaaggcagaaacggttcttattgttggaaggatcagtgaaaccatccaccaacacacttgtggaggaggcatggaacgcttcacccacacgattgttgagctcatagtagacaatagagcaccagtgttttggttcctcataagcaaccgcctgaacatctcctctgttgatttctgagggcaggggaggcgccatcatgtttgtgtccatcggctgagagccatcctgggtcatggggtcttcaggaggcaggtaagcaggtgggggcgtatcagctggcatctggaaagggcttcctgggtctgagctggtgggagagtgagggtaggtgctgctgctgctcccaggagagtttgggtaactgctattgggagagtgaggaaacgggtggctgttgggttgctggaaagaatctggaaaagtggcgttgagtggcatgtgaggctcattttgtcctaagttacggaactgagctaagaggctgtgctgaggattatattcgctgtgtcttggaaccagcacaggaggaagtacagggctttctactctcttatagtggtagggattgatgcagacctccttctgcttggaaccaaaaggaaactcacagcattccagtggttttagttcatggtggctctgaagatcgggccagcgccacacacggcagtaaatgacatgaggcagtcccttccggtgggagacttgcagcctgccatccagagagcggggaatggtgacacagttactcggttgccctgggcagctcaaggccttttccagttcctccatggcacctttctttttcttcagttttttcaccaaagcatcaacagctttctctgcccatttttcttcttcatcgccctgtttccacccaagaagtctcttcacagctggacttgtaaaggaaaataaacttgtcacattcataatgacagcactagttatactccttggatatggtgaaataaagctgtctccaaatgcaaaaggacagcagaagagatttgtttatttacagagaagtctctttaacttcttagtttgaagtccagaagagtagaaattaccattcctagtgtttaaaaaagtaacccagtcagcacgaaaaggatgctttctcaggagatggttctgagaccggcctcaattttcagaaggaacgcgcctttactggttatcttgcaccgtgtatttaaaaattgcatgctcttcaaaataaacaaaagctcagctactgtagctgtgagatctggcaggcatttgttcctcctcccctcctaaagcacatcaagaaaacgttctccctttaaagccttcatacagtttcagcaactagaaaaacaagcccacatctgtctctcacgcccaccacccccaccttcctacagaaacaaccccgagaaacactaacaaagacagggagcagagtaaaggaacagttgttcaaccgcgaactcacgaatacacatgcagtg

SEQ ID NO: 9529 - RNA, 2233 nt, Homo sapiens
  source 1..2233: mol_type = other RNA
agggtgtgtgtgtttttttttttttttgtttaaatttctgaatccaacagttggtcacagaggtcaagtattatcaaggctcctttgtcagttctcaatcgtgtctgactcatccatccttcaagtacatgcaaggctcaatagttttccagaggcagatgcctggggccatttaagatacagatgaaataggattatgaggtgaacccatttgagtaagaactttatccagccactggagggggccgtgcagatgtatctcaatccagcagggggtgctagtaacatcctggcggtggtattctgctccccagcccttcacaaagctcatacgtatagtacacatttttgtaagctcatagactgtctcaaatccatggttcacagactgtgccaataactgagcaaattcttggttgttaaaaattttcagactacacccactagggatcttgcaaacagtagtaggatgaaatccatgatggtagttgcagttccgactttgcacaaagatgctactgtcactaaggcattcggcatacacctcccctccaacataataaagatgaactccttttccaatatgccgcctggtgttttcaatagtggaattccggttaacattggagagcagcccaaggcagaaacggttcttattgttggaaggatcagtgaaaccatccaccaacacacttgtggaggaggcatggaacgcttcacccacacgattgttgagctcatagtagacaatagagcaccagtgttttggttcctcataagcaaccgcctgaacatctcctctgttgatttctgagggcaggggaggcgccatcatgtttgtgtccatcggctgagagccatcctgggtcatggggtcttcaggaggcaggtaagcaggtgggggcgtatcagctggcatctggaaagggcttcctgggtctgagctggtgggagagtgagggtaggtgctgctgctgctcccaggagagtttgggtaactgctattgggagagtgaggaaacgggtggctgttgggttgctggaaagaatctggaaaagtggcgttgagtggcatgtgaggctcattttgtcctaagttacggaactgagctaagaggctgtgctgaggattatattcgctgtgtcttggaaccagcacaggaggaagtacagggctttctactctcttatagtggtagggattgatgcagacctccttctgcttggaaccaaaaggaaactcacagcattccagtggttttagttcatggtggctctgaagatcgggccagcgccacacacggcagtaaatgacatgaggcagtcccttccggtgggagacttgcagcctgccatccagagagcggggaatggtgacacagttactcggttgccctgggcagctcaaggccttttccagttcctccatggcacctttctttttcttcagttttttcaccaaagcatcaacagctttctctgcccatttttcttcttcatcgccctgtttccacccaagaagtctcttcacagctggacttgtaaaggaaaataaacttgtcacattcataatgacagcactagttatactccttggatatggtgaaataaagctgtctccaaatgcaaaaggacagcagaagagatttgtttatttacagagaagtctctttaacttcttagtttgaagtccagaagagtagaaattaccattcctagtgtttaaaaaagtaacccagtcagcacgaatacacatgcagtgaggcaatcgactccggtaaagggaaaggaacgagacaccaggagacgcagcgggtgtaggcggaagagggggaaaaaattacgcgccgccgccaaacctttgaataaattagaggggatctcggtgcgaactttccttgacctcgaccccaaagaggcttgctggggccgagaagaaaacccgtgcgggatgtggaggggcccggggcgccggggtcccccgcccgcgagacccgctccaccaggcgccttggagagcagcgccagcggtcgtcctccagctcccgcaggggtcgccccgccggcgcgggggacacaatgggtccgcgggccacgcgaacgggcctcggcccggcggcagcacgggagagatgtgaggagcgcgcggaaggggagcgcggccggggagatcccagcgcggtcaggcccgggagccgaggctcgggggcccgggaactgggcttcccacagc

SEQ ID NO: 9530 - RNA, 36 nt, Homo sapiens
  source 1..36: mol_type = other RNA
agggtgtttctctcatctctcaagagcccccaaatt

SEQ ID NO: 9531 - RNA, 91 nt, Homo sapiens
  source 1..91: mol_type = other RNA
aggtagactgggatttgttgttgagcgcagtaagacaacaacaaaatcactagtcttccagatggggccagccggtccactctgtatccag

SEQ ID NO: 9532 - RNA, 2463 nt, Homo sapiens
  source 1..2463: mol_type = other RNA
aggtattgccaccctttctagtcagaggactggaggaaaaatgatgctatatgagatgccatagagccagagttgggtttacgtcctagctctgcctcttcttagcctgtgaccaagggcaaatgactctctgagcatcatttctttgtctccataaagagtttagcgcagtgcctggcagatggaagactatcactactcgatgtttgcaaactccaggaaccttgctctgcagggagatcactgtcagtggggagctgctcctctctccctttctgtgcctgtgcctctcattgcagtgattatgtagacagccttggaaacggggcagcttgggagttcagcactggcctctgcggtgccatggcaaccagcttcccagcaatcacccctaataatagccactcgagagctcttccacctgggcagaggctccccagggagttcgggcttctcttggagtaactgcacaaagctacctgttgggaacaaattatgagagggaaggagggaggggagagcatgctatctcagggggagagacgtgagaaaggaggcagacaagaagtctctagcctgtgatgtgtggagtgggcccaggggcctggggatgctgccattgggttcccggagcccactggctgtaggaatgtgtaattccacagtgggaggtagaggcccatggacacttttgccactcaccaaccttgcagagagtgaaagaccaaatatgagcgctcataaagccagccctcgctgttaccagatttcttcattaggctcctgtcgagatgctcactgccaactcatcatcttgtctggactgcagccgcctcccttacggctgcctgctggagagaatgtgctcagaggcctccttcaatcaatatctttccagaatgacagttctcaaaaaggcaccagtcccgcttggctaataaatgattattcctcttatctatccagtgcttcttgatcatttaaggctcagcttcttattaagtctttcttggtcataccagcccatttgctcctcacttctccccactatgaatttttggtctgtttttcctgtcctctgtgggaaaattgttggccgtttctctcactgggcaaaattattggatgtgtcttctgtatagtaaaaattactggctgcatctcaatcggcgaggcttttctctccaggggcaaaactgttgcctgcatgtctctgaaggaaaattgccatctgcctcactctgtaggaaaattgccagttgtgtccccattatggagaaattgtcaaccatgtctccaaacggaagaacgtgccagccgtgcttccctcaaagactggagcaccaggcaaggaagccgcagaagaagttgctatgaaggggagagcattcaatcaatgagatgtcttcagagttctcttacattagataaggtctctatattgggtagaactctacaaatggtttgatattctcttaaattcccccatacatacacacacttcattcaatatcccctaatgtctaagaatgtgggctttagagttggatggtcccagcttctgccactttacaggctgtgtggcctttagcaaattatttaacctctctaagactcattgccctcatcatctatcaaatggcaataacaattgaacctgactcctagaattgttgtgaagattaaacgaaacagtatacataaagaacttagaacatggtaagaattcaataaatcatagttattcaaatggctggcttctctgattcttatcaccagctgagtatggcaaaatatcaggacctactatgtagtgtttcattttgacaggtgcaagattcctttattcaagtcaataaaaacaacagtaagagcaacagcagcaacaccagctagtttactttttattgagcatatatctgccaggtcctgtaagacatctcttaaaatcttcctaagaagtctgtttcccattttacaaatatagaaagttagcctgaaagatgttaagcagcttgcacagctcatgcaaccaaagagggcagaatcaagatcctgagcctagagctcctaaccagcatgcctcacataaccaggatgctacgcgtaaccagcacactacacgtaaccagcatgccacacataaccagcatgctacacataaccagcatgctacacgtaaccagcatgctacacataaccaacatgttattcaatgaaacactagtcccatgagagaatcttcagggcaaaggggaaggggaagctctgtggtcataggaataggagaatgcccttgccaggagcatcacaatggacactagcataataatggctccaagaagtctttccatattccctatagggactagcacaggtttgagcactcagtaggctaccaataaaaagctctaaataatgccatccctgctcaaaaatattcagcccacaaaacagagaaca

SEQ ID NO: 9533 - RNA, 2367 nt, Homo sapiens
  source 1..2367: mol_type = other RNA
aggtattgccaccctttctagtcagaggactggaggaaaaatgatgctatatgagatgccatagagccagagttgggtttacgtcctagctctgcctcttcttagcctgtgaccaagggcaaatgactctctgagcatcatttctttgtctccataaagagtttagcgcagtgcctggcagatggaagactatcactactcgatgtttgcaaactccaggaacctttaagaaatggatcagtggattaggagcagtgttttcctgtagaaaaccagtactgggaacacagaggcagactgcctgatccatgagaagacagtgaagcagtgaccagctcacaccagggtccctccaggcagtgcttggcccatgccaagatgggctgtcgtactcagctgtgaactgctcaccttgctctgcagggagatcactgtcagtggggagctgctcctctctccctttctgtgcctgtgcctctcattgcagtgattatgtagacagccttggaaacggggcagcttgggagttcagcactggcctctgcggtgccatggcaaccagcttcccagcaatcacccctaataatagccactcgagagctcttccacctgggcagaggctccccagggagttcgggcttctcttggagtaactgcacaaagctaccagatttcttcattaggctcctgtcgagatgctcactgccaactcatcatcttgtctggactgcagccgcctcccttacggctgcctgctggagagaatgtgctcagaggcctccttcaatcaatatctttccagaatgacagttctcaaaaaggcaccagtcccgcttggctaataaatgattattcctcttatctatccagtgcttcttgatcatttaaggctcagcttcttattaagtctttcttggtcataccagcccatttgctcctcacttctccccactatgaatttttggtctgtttttcctgtcctctgtgggaaaattgttggccgtttctctcactgggcaaaattattggatgtgtcttctgtatagtaaaaattactggctgcatctcaatcggcgaggcttttctctccaggggcaaaactgttgcctgcatgtctctgaaggaaaattgccatctgcctcactctgtaggaaaattgccagttgtgtccccattatggagaaattgtcaaccatgtctccaaacggaagaacgtgccagccgtgcttccctcaaagactggagcaccaggcaaggaagccgcagaagaagttgctatgaaggggagagcattcaatcaatgagatgtcttcagagttctcttacattagataaggtctctatattgggtagaactctacaaatggtttgatattctcttaaattcccccatacatacacacacttcattcaatatcccctaatgtctaagaatgtgggctttagagttggatggtcccagcttctgccactttacaggctgtgtggcctttagcaaattatttaacctctctaagactcattgccctcatcatctatcaaatggcaataacaattgaacctgactcctagaattgttgtgaagattaaacgaaacagtatacataaagaacttagaacatggtaagaattcaataaatcatagttattcaaatggctggcttctctgattcttatcaccagctgagtatggcaaaatatcaggacctactatgtagtgtttcattttgacaggtgcaagattcctttattcaagtcaataaaaacaacagtaagagcaacagcagcaacaccagctagtttactttttattgagcatatatctgccaggtcctgtaagacatctcttaaaatcttcctaagaagtctgtttcccattttacaaatatagaaagttagcctgaaagatgttaagcagcttgcacagctcatgcaaccaaagagggcagaatcaagatcctgagcctagagctcctaaccagcatgcctcacataaccaggatgctacgcgtaaccagcacactacacgtaaccagcatgccacacataaccagcatgctacacataaccagcatgctacacgtaaccagcatgctacacataaccaacatgttattcaatgaaacactagtcccatgagagaatcttcagggcaaaggggaaggggaagctctgtggtcataggaataggagaatgcccttgccaggagcatcacaatggacactagcataataatggctccaagaagtctttccatattccctatagggactagcacaggtttgagcactcagtaggctaccaataaaaagctctaaataatgccatccctgctcaaaaatattcagcccacaaaacagagaaca

SEQ ID NO: 9534 - RNA, 2647 nt, Homo sapiens
  source 1..2647: mol_type = other RNA
aggtattgccaccctttctagtcagaggactggaggaaaaatgatgctatatgagatgccatagagccagagttgggtttacgtcctagctctgcctcttcttagcctgtgaccaagggcaaatgactctctgagcatcatttctttgtctccataaagagtttagcgcagtgcctggcagatggaagactatcactactcgatgtttgcaaactccaggaacctttaagaaatggatcagtggattaggagcagtgttttcctgtagaaaaccagtactgggaacacagaggcagactgcctgatccatgagaagacagtgaagcagtgaccagctcacaccagggtccctccaggcagtgcttggcccatgccaagatgggctgtcgtactcagctgtgaactgctcaccttgctctgcagggagatcactgtcagtggggagctgctcctctctccctttctgtgcctgtgcctctcattgcagtgattatgtagacagccttggaaacggggcagcttgggagttcagcactggcctctgcggtgccatggcaaccagcttcccagcaatcacccctaataatagccactcgagagctcttccacctgggcagaggctccccagggagttcgggcttctcttggagtaactgcacaaagctacctgttgggaacaaattatgagagggaaggagggaggggagagcatgctatctcagggggagagacgtgagaaaggaggcagacaagaagtctctagcctgtgatgtgtggagtgggcccaggggcctggggatgctgccattgggttcccggagcccactggctgtaggaatgtgtaattccacagtgggaggtagaggcccatggacacttttgccactcaccaaccttgcagagagtgaaagaccaaatatgagcgctcataaagccagccctcgctgttaccagatttcttcattaggctcctgtcgagatgctcactgccaactcatcatcttgtctggactgcagccgcctcccttacggctgcctgctggagagaatgtgctcagaggcctccttcaatcaatatctttccagaatgacagttctcaaaaaggcaccagtcccgcttggctaataaatgattattcctcttatctatccagtgcttcttgatcatttaaggctcagcttcttattaagtctttcttggtcataccagcccatttgctcctcacttctccccactatgaatttttggtctgtttttccctctgtgggaaaattgttggccgtttctctcactgggcaaaattattggatgtgtcttctgtatagtaaaaattactggctgcatctcaatcggcgaggcttttctctccaggggcaaaactgttgcctgcatgtctctgaaggaaaattgccatctgcctcactctgtaggaaaattgccagttgtgtccccattatggagaaattgtcaaccatgtctccaaacggaagaacgtgccagccgtgcttccctcaaagactggagcaccaggcaaggaagccgcagaagaagttgctatgaaggggagagcattcaatcaatgagatgtcttcagagttctcttacattagataaggtctctatattgggtagaactctacaaatggtttgatattctcttaaattcccccatacatacacacacttcattcaatatcccctaatgtctaagaatgtgggctttagagttggatggtcccagcttctgccactttacaggctgtgtggcctttagcaaattatttaacctctctaagactcattgccctcatcatctatcaaatggcaataacaattgaacctgactcctagaattgttgtgaagattaaacgaaacagtatacataaagaacttagaacatggtaagaattcaataaatcatagttattcaaatggctggcttctctgattcttatcaccagctgagtatggcaaaatatcaggacctactatgtagtgtttcattttgacaggtgcaagattcctttattcaagtcaataaaaacaacagtaagagcaacagcagcaacaccagctagtttactttttattgagcatatatctgccaggtcctgtaagacatctcttaaaatcttcctaagaagtctgtttcccattttacaaatatagaaagttagcctgaaagatgttaagcagcttgcacagctcatgcaaccaaagagggcagaatcaagatcctgagcctagagctcctaaccagcatgcctcacataaccaggatgctacgcgtaaccagcacactacacgtaaccagcatgccacacataaccagcatgctacacataaccagcatgctacacgtaaccagcatgctacacataaccaacatgttattcaatgaaacactagtcccatgagagaatcttcagggcaaaggggaaggggaagctctgtggtcataggaataggagaatgcccttgccaggagcatcacaatggacactagcataataatggctccaagaagtctttccatattccctatagggactagcacaggtttgagcactcagtaggctaccaataaaaagctctaaataatgccatccctgctcaaaaatattcagcccacaaaacagagaaca

SEQ ID NO: 9535 - RNA, 2651 nt, Homo sapiens
  source 1..2651: mol_type = other RNA
aggtattgccaccctttctagtcagaggactggaggaaaaatgatgctatatgagatgccatagagccagagttgggtttacgtcctagctctgcctcttcttagcctgtgaccaagggcaaatgactctctgagcatcatttctttgtctccataaagagtttagcgcagtgcctggcagatggaagactatcactactcgatgtttgcaaactccaggaacctttaagaaatggatcagtggattaggagcagtgttttcctgtagaaaaccagtactgggaacacagaggcagactgcctgatccatgagaagacagtgaagcagtgaccagctcacaccagggtccctccaggcagtgcttggcccatgccaagatgggctgtcgtactcagctgtgaactgctcaccttgctctgcagggagatcactgtcagtggggagctgctcctctctccctttctgtgcctgtgcctctcattgcagtgattatgtagacagccttggaaacggggcagcttgggagttcagcactggcctctgcggtgccatggcaaccagcttcccagcaatcacccctaataatagccactcgagagctcttccacctgggcagaggctccccagggagttcgggcttctcttggagtaactgcacaaagctacctgttgggaacaaattatgagagggaaggagggaggggagagcatgctatctcagggggagagacgtgagaaaggaggcagacaagaagtctctagcctgtgatgtgtggagtgggcccaggggcctggggatgctgccattgggttcccggagcccactggctgtaggaatgtgtaattccacagtgggaggtagaggcccatggacacttttgccactcaccaaccttgcagagagtgaaagaccaaatatgagcgctcataaagccagccctcgctgttaccagatttcttcattaggctcctgtcgagatgctcactgccaactcatcatcttgtctggactgcagccgcctcccttacggctgcctgctggagagaatgtgctcagaggcctccttcaatcaatatctttccagaatgacagttctcaaaaaggcaccagtcccgcttggctaataaatgattattcctcttatctatccagtgcttcttgatcatttaaggctcagcttcttattaagtctttcttggtcataccagcccatttgctcctcacttctccccactatgaatttttggtctgtttttcctgtcctctgtgggaaaattgttggccgtttctctcactgggcaaaattattggatgtgtcttctgtatagtaaaaattactggctgcatctcaatcggcgaggcttttctctccaggggcaaaactgttgcctgcatgtctctgaaggaaaattgccatctgcctcactctgtaggaaaattgccagttgtgtccccattatggagaaattgtcaaccatgtctccaaacggaagaacgtgccagccgtgcttccctcaaagactggagcaccaggcaaggaagccgcagaagaagttgctatgaaggggagagcattcaatcaatgagatgtcttcagagttctcttacattagataaggtctctatattgggtagaactctacaaatggtttgatattctcttaaattcccccatacatacacacacttcattcaatatcccctaatgtctaagaatgtgggctttagagttggatggtcccagcttctgccactttacaggctgtgtggcctttagcaaattatttaacctctctaagactcattgccctcatcatctatcaaatggcaataacaattgaacctgactcctagaattgttgtgaagattaaacgaaacagtatacataaagaacttagaacatggtaagaattcaataaatcatagttattcaaatggctggcttctctgattcttatcaccagctgagtatggcaaaatatcaggacctactatgtagtgtttcattttgacaggtgcaagattcctttattcaagtcaataaaaacaacagtaagagcaacagcagcaacaccagctagtttactttttattgagcatatatctgccaggtcctgtaagacatctcttaaaatcttcctaagaagtctgtttcccattttacaaatatagaaagttagcctgaaagatgttaagcagcttgcacagctcatgcaaccaaagagggcagaatcaagatcctgagcctagagctcctaaccagcatgcctcacataaccaggatgctacgcgtaaccagcacactacacgtaaccagcatgccacacataaccagcatgctacacataaccagcatgctacacgtaaccagcatgctacacataaccaacatgttattcaatgaaacactagtcccatgagagaatcttcagggcaaaggggaaggggaagctctgtggtcataggaataggagaatgcccttgccaggagcatcacaatggacactagcataataatggctccaagaagtctttccatattccctatagggactagcacaggtttgagcactcagtaggctaccaataaaaagctctaaataatgccatccctgctcaaaaatattcagcccacaaaacagagaaca

SEQ ID NO: 9536 - RNA, 1704 nt, Homo sapiens
  source 1..1704: mol_type = other RNA
aggtattgccaccctttctagtcagaggactggaggaaaaatgatgctatatgagatgccatagagccagagttgggtttacgtcctagctctgcctcttcttagcctgtgaccaagggcaaatgactctctgagcatcatttctttgtctccataaagagtttagcgcagtgcctggcagatggaagactatcactactcgatgtttgcaaactccaggaacctttaagaaatggatcagtggattaggagcagtgttttcctgtagaaaaccagtactgggaacacagaggcagactgcctgatccatgagaagacagtgaagcagtgaccagctcacaccagggtccctccaggcagtgcttggcccatgccaagatgggctgtcgtactcagctgtgaactgctcaccttgctctgcagggagatcactgtcagtggggagctgctcctctctccctttctgtgcctgtgcctctcattgcagtgattatgtagacagccttggaaacggggcagcttgggagttcagcactggcctctgcggtgccatggcaaccagcttcccagcaatcacccctaataatagccactcgagagctcttccacctgggcagaggctccccagggagttcgggcttctcttggagtaactgcacaaagctacctgttgggaacaaattatgagagggaaggagggaggggagagcatgctatctcagggggagagacgtgagaaaggaggcagacaagaagtctctagcctgtgatgtgtggagtgggcccaggggcctggggatgctgccattgggttcccggagcccactggctgtaggaatgtgtaattccacagtgggaggtagaggcccatggacacttttgccactcaccaaccttgcagagagtgaaagaccaaatatgagcgctcataaagccagccctcgctgttaccagatttcttcattaggctcctgtcgagatgctcactgccaactcatcatcttgtctggactgcagccgcctcccttacggctgcctgctggagagaatgtgctcagaggcctccttcaatcaatatctttccagaatgacagttctcaaaaaggcaccagtcccgcttggctaataaatgattattcctcttatctatccagtgcttcttgatcatttaaggctcagcttcttattaagtctttcttggtcataccagcccatttgctcctcacttctccccactatgaatttttggtctgtttttcctgtcctctgtgggaaaattgttggccgtttctctcactgggcaaaattattggatgtgtcttctgtatagtaaaaattactggctgcatctcaatcggcgaggcttttctctccaggggcaaaactgttgcctgcatgtctctgaaggaaaattgccatctgcctcactctgtaggaaaattgccagttgtgtccccattatggagaaattgtcaaccatgtctccaaacggaagaacgtgccagccgtgcttccctgaaatgtcccgtgtgcctgcgtttcatcattcccactggaatgcaggcttcacgagagcaggggcttccctctggttcacaactgctcctccatagcacatagtaggagttcaaggagtatctactgagtgaatagatggttagatggttcctgggttagtgcttctttgagcaaatggagtaaagg

SEQ ID NO: 9537 - RNA, 57 nt, Homo sapiens
  source 1..57: mol_type = other RNA
aggtattgccaccctttctagtccctattagactagaaagggtggcaatacctcttc

SEQ ID NO: 9538 - RNA, 63 nt, Homo sapiens
  source 1..63: mol_type = other RNA
aggtattgccaccctttctagtctaatagggactagaaagggtggcaatactcttcaaaaact

SEQ ID NO: 9539 - RNA, 570 nt, Homo sapiens
  source 1..570: mol_type = other RNA
aggtctgcattcaaatccccagagacttagttccagaagcttccaacaatgcccttaggatgtatgactaggtctgaacattcagtaaagtgtgagcttgtggcagtctctgtatatagactcagttatctgcattcatctgtctcttttcctaggtcaggagagtcccaagaagaaggatcatatctggtttcctcttctgcctctccccatggtgtctaggagagtgcacactcagtcagcattgataactaactctgatacattcaggaggaggaaaaggggtatctccattccaaagcactttcttctttgccctccctgcatgggaagtctttggggtcatttctaccagtggatggaacctcaggccagtttgcttcccaccacacacagaccctatgtgatcctggaactttgaaaaagttatttatgtgtccatgcctcagtcttctcatccgatttttcccactctgggttacagaggcttgactctacttgtccagtatggttcacctggaaactggatatccagtgaggagaggagaaggggctgtcagaaaatcagct

SEQ ID NO: 9540 - RNA, 482 nt, Homo sapiens
  source 1..482: mol_type = other RNA
aggtctgcattcaaatccccagagacttagttccagaagcttccaacaatgcccttaggatgtatgactaggtctgaacattcagtaaagtgtgagcttgtggcagtctctgtatatagactcagttatctgcattcatctgtctcttttcctaggtcaggagagtcccaagaagaaggatcatatctggtttcctcttctgcctctccccatggtgtctaggagagtgcacactcagtcagcattgataactaactctgatacattcaggaggaggaaaaggggtatctccattccaaagcactttcttctttgccctccctgcatgggaagtctttggggtcatttctaccagtggatggaacctcaggccagtttgcttcccaccacacacagaccctgctgccattcttttccagggcccagaacaatcccaggggccttaactacagactctaattgggcgcatcagcatcacgagt

SEQ ID NO: 9541 - RNA, 453 nt, Homo sapiens
  source 1..453: mol_type = other RNA
aggtctgcattcaaatccccagagacttagttccagaagcttccaacaatgcccttaggatgtatgactaggtctgaacattcagtaaagtgtgagcttgtggcagtctctgtatatagactcagttatctgcattcatctgtctcttttcctaggtcaggagagtcccaagaagaaggatcatatctggtttcctcttctgcctctccccatggtgtctaggagagtgcacactcagtcagcattgataactaactctgatacattcaggaggaggaaaaggggtatctccattccaaagcactttcttctttgccctccctgcatgggaagtctttggggtcatttctaccagtggatggaacctcaggccagtttgcttcccaccacacacagaccctggaaactggatatccagtgaggagaggagaaggggctgtcagaaaatcagct

SEQ ID NO: 9542 - RNA, 340 nt, Homo sapiens
  source 1..340: mol_type = other RNA
aggtctgcattcaaatccccagagacttagttccagaagcttccaacaatgcccttaggatgtatgactaggtctgaacattcagtaaagtgtgagcttgtggcagtctctgtatatagactcagttatctgcattcatctgtctcttttcctaggtcaggagagtcccaagaagaaggatcatatctggtttcctcttctgcctctccccatggtgtctaggagagtgcacactcagtcagcattgataactaactctgctgccattcttttccagggcccagaacaatcccaggggccttaactacagactctaattgggcgcatcagcatcacgagt

SEQ ID NO: 9543 - RNA, 330 nt, Homo sapiens
  source 1..330: mol_type = other RNA
aggtctgcattcaaatccccagatgttgtgaactggcatgtgagatttacattagaaggcctttctaaagtgatatttttttctactggcatactagaatgttcagtcagtgatatgttatgactctccaaggaaaagttatttgccattatttcttctctgagaggtggacttgtaaaaggcgaatccaagttgatgctgatccccactgttgcttttgctttcaaaattcatctcagagtattgcagttctgagaacctctgcactcctggggaattctcactctgtcgctcaggctggagggcagaggcacattcacggctcactgc

SEQ ID NO: 9544 - RNA, 436 nt, Homo sapiens
  source 1..436: mol_type = other RNA
aggtctgcattcaaatccccagatgttgtgaactggcatgtgagatttacattagaaggcctttctaaagtgatatttttttctactggcatactagaatgttcagtcagtgatatgttatgactctccaaggaaaagttatttgccattatttcttctctgagaggtggacttgtaaaaggcgaatctggggcactgccgtccgccgagcttgggcgcgcggcagcgagaaggcactggaggaggagcagccggggcgtacgcgccctggcctccagcaggccggggagggcgcgcatggcgccagagggtccgcctgggtcctcgtggagactgctccctcagctcgccgccgcgggtgtccagagtccctgcgcacactcgcaggtggcccggcgctcgcagccagtgccgcgggtaggacgctgaagaaaag

SEQ ID NO: 9545 - RNA, 529 nt, Homo sapiens
  source 1..529: mol_type = other RNA
aggtgctccaggctggctcacaaacttcctgggcctcggtttccacatctgtacagggccgggctggctcacaaacttcctgggcctcggtttccacacctgtacagggccgggctggctcacaaacttcctgggcctcggtttccacatctgtacagggccgggctgacttcacaaactccaaaaagctgcaggactctcttcatcttcagaataaatgttgagggctccctcatgcttccgtctctccatgagggatcaaaggaaactcctccacaagttccagtgaaaacactcatgaagctcctgcagctgctcctcaggacggggcgagaggaaggacttccacattccaacgatttgagctggaccccaggttgcacagctaaggctgaagagaagccaagtctctcgggtgatcaacgttcaacggccgggtgcggtggctcacgcctgtaatcccagcactttgggaagctgaggcagatggatcacctgaggtcaggagtttggcagcgggcgcctgtag

SEQ ID NO: 9546 - RNA, 1667 nt, Homo sapiens
  source 1..1667: mol_type = other RNA
aggtggatgcaatgtgacctcagacaactggtgccatggaggggaaggaagctggcttgtagcaggtctctcagaggcaggaagttgcggggagtcagagccattgtctacagaggcggggacactgaatgaccctggaatcctttgacccccttccctcagccccttcagcggggcaggaagcggatctggtatgttgggggtattttgcccacaccacactcctggggtgtcagatcgatgtcttctggggccacggggctggccatggagaagttctggaggatggtggtgaagaagaggaacaattccgcacgggcgatgccttcaccaagacaaatccgcttccctaaggagaaggggataaaagcttcagtctttttcagtgccccattggcatccagaaagtggtcaggattgaaggcgtctggtttttcaaagtagtgtgggtcatggagagcagtgctcaggatgagaaatacttctgtgtccttggggatgatgtaccctcggaagctggtgtgttgggtgacaatgtggggcacacccatggggagaaggtcggaaaatctctgaatctcatagatgactgcctctgtgtatggcattttggctcggtcatgaagctctggagggcgatgtgggccaatcacctgttcaatctccctgtagactctctctgcaacatgagggtatttgagcatgagcaggaagccgtagcggagagtggtgctggtggtctcagtgccagcaaagaagagcgagagcgtgttgaggttgaggttctggtggctgaattcactgtgtgcgttggatttctctttttccatgtggagcaggtaggtgtcgatgaggtccttgggggcgctggggtccagggtttcacggtgcttctccacactgtggccaatgtaagcattgatttcctgcaggtttttgtaaacttgcctgtgtgccccaggaaagtatttcaagaagccagagaagagctcaaacagctggccgaatacagagctgatgagtgaaaaagtctggtagaacaagttcagcatcttcaggaactcttgatcttggtagtggaatcgttttccaaagacgatggagcagatgatgttggcggtaatggactggaagaggaaggtggggtccatgagggcccccttggatttccgaagctcctctatcagacactgagcctcctcctgaatccgctcctccacactccgctttcccatcccgaagtccctcatagtggtcacagagaatcgccgaagcaccttccagcggtttccattggcaaagatcacaccatatccccggaagaatgggtcgaccatggcgatttttccccggccagagaaggcctcagccttgtccacaagggcctcccgtatggcctctactccacacagcatgaccacgggcctcggtcccaggtgtaccgtgaagacgtccccatatttctctcggaacctcagaaaggatttgagtaggcctcttctatccatctgcagaaggtttcccaaaaggggcagagggcggggccctggtgggaggcggtcatgggtgttagggtggcgctgaaccaggagtagcaagagtcctgtgaggagtgcaaggaagaggaggacgctgagttccatggtcctggtctgactgccctgcac

SEQ ID NO: 9547 - RNA, 773 nt, Homo sapiens
  source 1..773: mol_type = other RNA
aggtgtgtctgtagagtcctgactgcgtgccaggggctctgtctggcacatttctgaactttgcaaaattaattgtgccgaagagaacaccatcaaacgcgtccggcatacagcgtaaacatcttcagaccgtgattctgcgccatcaaacgctctccagctaatttcatttggtgattactctgctagaaaaccgaggccaagtgaaactgcggaaatgggaacaatgtacggaggaaaaatctcaccccattaagagatccgtttcttctccgcacaaataagcccaccccgcctccgaggcaagactagatggctccaggatactctcggcgcgcccgctggccatctcgggcaggggagccccacacccggcaggaggaccaggacgcgagcggcggcgcctcggccctgggctgtttaggtaattcgcaaagtcccaacaatcatccccctctcccagaagctggttttcttgtgtgcagtggttacagaggcggcgaaaacacggttccccgctttcctctcctcaaggcactgtttgcagcggcagcagcggccgcattcggggaggcgcggtcctccccgcagagccgtcgcgcactcggcctttctcgaggatttgcctgggctcggccgcctcgctctcccctgcgcttccatgaccttctgagagcggcctcaccaccggaggctcggaggaagcaccaccctcggcgtccggggcccgtcgcgcggccgcgttcctccgactccttggagcacccgcgcgc

SEQ ID NO: 9548 - RNA, 505 nt, Homo sapiens
  source 1..505: mol_type = other RNA
aggttgcctgtgaggtgttcagacttcctacacagcaattgcttccaagagggcaagggggcctcactggaaacaggcaattctgcttccggccaattctgccacattcttccaactgaggttgcatgttcactgaccaacagaccagctgtagcaagggacatatgcaagaccacaggagacggtcacagcaagctggtacagcacagaaaacagacgggaccctagtctggccgagcatgggctggtgaggctgtgtcagctcctgctatgacatgtcacttgtgttgatggttcttttactttagtgtcttctgggtttcaaagcttatatttccagaacagtttagacttcacaatgaagatcactccttctaaaacatgacccttccagggcaagccattctcactccaccatgaagcacttatgccaaagcctggcttcttttcttttctcttgaatgcatgtcagtggcctccctgggctcgccgtctatgccaccct

SEQ ID NO: 9549 - RNA, 1584 nt, Homo sapiens
  source 1..1584: mol_type = other RNA
aggttgcctgtgaggtgttcatagccaacattcacagcagctgggggatggtgcactgcctagtcaaggagatctgggtagagcaccaacagaatccactgctcctggcttgggtaaggtgtccactcaagagcaattagccattgagagagaggcaaaaccttgaagtctagacatggcagcagggctatttccagaggaaagtgtacaagagtgatgggaagttataccaaatggtgtccatagtacccacttgaataacttctactgaaaatgctctcctggccagtatgtacaactggccaggtgtttcttcctcagtaagaagagtatttcccaggcacttaacataatctcctttttttttgtttttctcacgtcagtcaggtaatatgtcaacatggtaacaaggttcgagggtggctcatctcacacgtgggcaggaacacccaatcatcatgctcatgaactacaaaaggatcatctctgtttttttaaaaatctctcaaacattgtttattatacaagtaaaccccaattctcatgatgggcttattggtaggatttctggtagcaagcatgggtaccagcgtctcttaattttttggattagtggtggtggaggtcagccaccagcaggatctggtcgtactgtatgaggatgtctttgatctttgtctttgatctcctccttggaaaactcatccatatacttctggtaataggacaccagggctttgaggctggactgatggatagcatatatctaggccatgtgatcaccacccttcacatggacacgtccatgccagcaaatcactccttgtctggaagcagaactggttccagcagctcatatattggtatgtatagctcgatcatctccaggggccgcctgttcaccttgattgctgcgtttgcagtgtgccacagctgtggctgtcttcttgcatctgaagacccgccggcccagggctcagctcgccgtgtgacagccccgggtactttgcccagcggggtgcaagcccggaccgcggcaagcgccactcccgggcagtcgcggccacaactgcttccgggtgagtgggtcgtcgaccctgtggccccgcccatccttcgcctcctcagtcggccgctcaggctgcggctcctcccggggccggttcccgctgtctcagccgcggcgcagagggcacatcggcctgaccgactagccggctgccagtgccgggagccgccgcgtccatccccgcccgcctggccggggacccaggactgagtcgtccagctgcgcccctcgcccatagccccagcgggcgccgggcgggcgagcagctcttcggcccttcccggacagcgacgcagtcgcagcgcgcgccctaacacaggtaagggccgctcctcccgccagcccggtgggagcagggagcggggagttgggaacctttttcccggcctccgcagtcccgtgggatccgcgccgcctccgacctcggctagggggccgggcttccctggggactggccggcccgcggcgggctcccgggctggggtcgccccctgcctgcggcgttctcagacat

SEQ ID NO: 9550 - RNA, 1126 nt, Homo sapiens
  source 1..1126: mol_type = other RNA
agtgcctgagggagtaagagccccatccctgaaggtacacaagttgtggcagcaaccatctggcctgcagtttccagaggggagtcaggcgtggggtgggactggagtgaacgggtagatgcttccacatgcggcagttggcactgacggcaggaacacgggggtggcttaatgggtcctggggctcccctctggccctcaggaaggcaggagcatgaggggcttgggatgcagcacctgcaaatttgcacgttcctggcctcaggaggcctccagtacagaaaagaccatcaacgaagctctgcagccatctgctaagaaacgccacagggaggggacagcatggccagccggggtgccatcaggctttgggtggggatcctggaggatcagacccatctaggtgggagcgctggggtgcaacccctagaggaggctgcaggcgcgcttctgctgccgcgtgggctgagggcacagcacggcccggatggcctcgtcgaacacggttttcaggcctctctgggtgagagctgagcactccaggtatttcaccgagtcaatctccttggccagtgccaggccctgcgggtaggtgatgggagccagcttcttctccttcagtttctcgatggtgtccttgtcgtcccgcaggtccagcttggtgcccaccaggatgatgggtgtgctggggcagtggtgccgcacttctgggaaccacttggcgcggacgttctcataagaggctgggctgacgagggagaagcagatgaggaagacgtccgtctgtggataggagagcggccggagacggtcgtagtcctcctgcccagcagtgtcccacagccccaggttcactggcttgctgtccaccatcacattggctgaatagttgtcaaacacggtggggatgtactctccgggaaaggcgttggtggtgtagctgatgagaaggcaggtcttgcccacggccccatctcccaccaccacacacttgatggcctgcatcgtgtccggagcctggagagtgtcggtggtgacagctcagggccaggcgcgtttctgcgggcgcaaggggtgtggaggctggtgaggcgcctgctgaggagcagcggtggtggggcaggag

SEQ ID NO: 9551 - RNA, 76 nt, Homo sapiens
  source 1..76: mol_type = other RNA
agtgcctgagggagtaagagccctgttgttgtaagatagtgtcttactccctcaggcacatctccaacaagtctct

SEQ ID NO: 9552 - RNA, 76 nt, Homo sapiens
  source 1..76: mol_type = other RNA
agtgcctgagggagtaagagccctgttgttgtcagatagtgtcttactccctcaggcacatctccagcgagtctct

SEQ ID NO: 9553 - RNA, 1972 nt, Homo sapiens
  source 1..1972: mol_type = other RNA
agtgcctgctatgtgccaggcacaatgtggcactcttacactcttgagagcaagagtaaccagaacaattatggttcctgccatcatgaagtttacagtctagtgaagaacccagacatcagatacttataaatagataattaaatgattacagttctttgaagtggtttggaggacaatcacagtttgctgtatggactaaatttaaaccagggaccatgaaaagggctccagaggaagtgacatttaaggtgagactgaagtttacattggagggtttgagacaggagggggaagagggaggggggagaggacagtgatccaggcagaagttctgaaaccagccagcgcgggtatgtttgaggaactgaaaggccaatgtggctggaaagaagataaagtgagactgtgatggtcagcatgggccagatggtgcaagacttacgggcaagtttcctcagccagaaactctctccctcattcatggcctcaggaatgacccctggttggggctcagagaatgataccccaaagtatggtgctttagtattgtttctgagcaaataggctcactgcctgatgcacatagaagccaatactatggtaccagcttttgagaacagaaaggctttattgcagggccacccagcaaggagactggaggcatggctcacatctgtctcctaatttggggtctggggcaagatttaaggggtcagagggtgatatggtttggctgtgtccccacccaaatctcatcttgaattctcacatgttgtgggagggacccagtgggagataattgaatcataggggcaggtctttcttgtgctgttcttgtgatagtgaataagtctcatgaggtctgatggttttgagaaacaggagtttccctgtacaagctctttgtttttgcctgctgccatccatgtaagatgtgacttgctcctccttgccttctgccatgattgtgaggtttccccagccacgtggaactgtaagtccaattaaacctcttttgtaaattgtccagtctcaggtatgtctttgtcagcagcgtgaaaacagactaatacagatggcaaggaaacgtattaggaattttggcttggcagggtctgattggagggtgtcaaatttgactacacgggtatgttgaggtggattttacccctggatctttctggtcaacagaccctttgctcctgaaagagttccagcatttaggttccgatcatgtctaggtcttcttggtaccacagggaggaatcattggttctgggtgttgttagatgtcaaagcattttctattgggcatgccctactgacatgacttggagttttggctctgtcataccttaagtcccagctactccggaggctgaggcagaaggatcacttgaggccaggagttccaggatgcacctgtgatagccatgattgctatgaccgcacctgtgaatagccactgccttccagcctgggcaacattgccagagtccgtctcttaagaaaaaaaaaatctttgaactaagtttgttgtgattttgtcttttgacaaagaagaaagggcaatgtgaattgccccaaatcacagagcgaaatggtagtagtcaggaccaaaacactttcttagccgttttcttagttcttgtacccatctgtttctgtattttcttcaccaggccatccagcagtgtctcttaaagggtagcccgagaaacaactgacttagaaaagcgtggggcacagtctgtctacgcagacccgaggaatctgcattttaacaaactcactgggaaattctcgcgcacgccaaggtttcaaagaccagggtcccgtggcacagtgccgcacagttgtcaaaacaagtgctgtccaattgttttggttttaaattctcactgcgtcatgggaaatgtagtttcgagcctcctctctcccgacgccccagccaatcctccggcgcttt

SEQ ID NO: 9554 - RNA, 682 nt, Homo sapiens
  source 1..682: mol_type = other RNA
agtgcctgctatgtgccaggcagggtactaggtgctgggaacaaacaggtgaacaagataaacacagttctgccctcctaaagcttacagtccagttagaggaacagacaaacagtccaacaagacaacaatccccagttgtgataagtactgaaaaaataactaaaaggctgatgtgagaatgactggaaacacctttttgtgttagggtaactcggaaaggcctctctaggtatggcactggtgctgttatgctgagagtatgcattccggataggacacgatgaaatggcacttcgcatcctcccaaccttagatttccatttagatgaatgtgcttctgtcctgagaagaagtgtccagccccagcttcatctaatgtttccaggtaatccttaacagccccaaaactgactccaaagaaagcaacacagtcaaactgtctgtccctctctcaggacaacgtcaataatatacccactttgggtatttggaatataattgcaaacttcagcctgaggccaataaaactttttatctagcttccatacttgggtcaatcctgcttcgtggctgttctctggatcctaaccgacatgctcagctccatgttaggagttctggaccactgtcttttgccctctttccttactaaaatgctctctggccaggcatggtggct

SEQ ID NO: 9555 - RNA, 3941 nt, Homo sapiens
  source 1..3941: mol_type = other RNA
agtgcctgctatgtgccaggcatgttgtaggcaattttcatgcatttgttcatgctatttccagtgcatggaatgtcctgcccaaaatctgtttcctggaaaatatccacccatctttcaagtgttggtacatggtttgtataaatttggtcatatctgtctgtctcactttctgttccttcagtcagtcagctttatgcaaatgtcaactgcagaaagtcctaatacaattatgtctactgggccataaactctgaggaacaggtccatgcctcattcatcatttcatccctaacacctgcctagtatctgacacttacattaattcatcttagccccaattagtcctattcttctttcatctgtgacaaagaataaaataagcatgaaaaaacttcatcagacactactaggttatcatttcagaaatcagaatagaaatacataaatataagaaacttgcaggagcataaggatgaatcttaatggatgaagcccagagaattcatgaacttcctcaagttacgagacacattaatggctcagggtttcttcttctttttttttttttttttttttttttttttttgagatggagtctcactttgttgcccaggctggagtgcagtggcgcaatttccactcactgcaagctccgcctcctcggttcacgccattctcctgcctcaacctcatgagtagctgggactacaggcgccggccaccacgcccagctaattttgtatttttagtagagatggggtttcaccgtgttagccaggatggtctcgatctcctgaccttgtgatcctccctccttggcctcccaaagtgctggggttacaggcttgagccaccgcgcccggcctcagggtttcttttataactgtgatcaggaagatgtgcttttctttctacttggttaagcaactaatcaaactcagcacaacaaaacaaagattctccttttctcccaagaagttcaacagttctagcgttgtagaacatttcacaaataaaaccatcctagtttccttttcccataaacagttgaacacatcagtgtgataagatcacctcacactatttcttggcttaatgctagcattgcctcctgcatacagatttctcttacccttctagcagatttaattgcttcttcccctgtattcccacagcactgtatatactctattatagctagtttacgaataataatattaattctggaccataaaattgcaactggtcaatgcctggcatataatgaacactcaaatgaacaaggaattgaatcttgctttaatgaagtaagtcaagactaattatgtcagttccaatcttaagaacgtccttggcttttaatgaggggtcttcatctttgaacacagatttagtttcagacagtggtttttgctgcctgtaataactaaagtttgcaaaaaaattaattatttgaggacactatatttttaagaaatgaatttccttaaactattcctacaagggtaatatacagtaagtgaaaaaccactaacacggtagttctcatagtggttgcttttatgtatgcatacttaagataattttaagtggttagaataggtccagagaacacctatattctatggtgttgccatttaatgttttaattatttaaaatacttaaataatttaatatttaatttgaaaaattaaatactgagtttgttgtgggcaaattagtggtgataaaacattattaatctaaaatctgctcttaaaatttgttcagattatcattgactgattggccccgccctccccatattcactcataatatgatttgttattttgtgattcttgacagttaagaaagcaattttaatacctgaaatgcaagtctagctgtggcttcattttaagaatttggtaattttgtaaaagtgcttgaatgcttgttttaccattgttatatctcaattcttataagaccctcagcagaatcaatttacatgactggcagtactaagccactttaaaattattttaaataattttatttgcttgggttctacttgtttgggttttacatactactgtggcatccttcttttaaggatataaactataattagaaatgatatggaaaaaagtgactagaaaacaaatctgaaggcttttaaaaatttcagagtacattagtaaatgctttaaaagacaacccatccaataacatatatgcaagttaacactacaaattcaatgacataagaaaatagattggacttacttttacattcacctctacagatactctataatgaacacactagtatgatgataataaagcaatcaagaacaatttatctctcagtctgtgtatatgtgactatctacatatttatttcacacacacatgccaaatacccacataacttcaatcctatatccatttacctctcagagtgatttaaagtagccacagtggcacataaaaggaaaaaaataatgaattccaggcttcctagtaagtaaagccaaatcaaattgttcaagtgatactatagtgctatttttacaggaaaacacagatttctataatttctggtcatttacttcatcattaaagtactatttgccaatattggtttcacataatgacaataaaacattcttgacttatatactacatgaaaaaaatagattatgagcttattttttgaccagtcatcaaacatgttttcatttgaataaagaaaattcttccagtttaatatgtttatcaatttgttttttcaatgaaacaaagtaaatttacagtaaagttactggtctcaatataagtcttccaatcttcaaattcagccgaacagtacaaggattacaggagaaaaaaaaacacaattaatctcttgtggctatcattttaggggctggttttctcatattgctgaattctaccacaccctgtcgtatttccaaggtttggatggtgctttaaatctgaactgcctgagaagattcagaaagcctttgttcttgggcttacacagtaagcactttgcgtgattcctaatcacatttttatccagaacacagtgttacgggtcacatttttctcaataatgcttatattgattgatgctctataaatataaacatatttacatacagaatacacacactgacatgggggtatgaagttagccagccatccataggaagaatggaataaaaattgcaggaagggtagtgtatgataccaagcccgtacagactatagacgccaatcccaagactgctgaagcaagaacacttctctgatcacgaataattatcttcacagtctcacaaaacttgtcggactggggactgatcggggtgccatatctgcagtaggtcacgaagtgctcgcagttgttccacagcaggctgtagggggtaaagcccagcagcttttcagccctccgcgccacctcctcgttgagcagtgcctttttctggagggactcgtccaggtgattgaccaggatgttagctccgtaggcgaagtcctccactgtgtccacgcggatgctggccactttgacaataacgcccaggatgagacgcttgttggagaccaccttctgcgtgcgccccatgtcgtctgtcagggccaacaggatgtcgggcatcatgtgggcaacacggttgtctcctaggtagatgccatagtgggtcaggtgggtccggggcacctccagcacgtcgcctcggtggaaagagctggtttcataaaaactgttcctccctttgtcttcgcccgcggcgcccgaactaaagagcgtgaagttggagatgaggagcagcttctccagtagtaaagacaccacctccagcatggggttcttcatccctgagtagctggagagacctctggtttcccggaccgttaagaaaggtggctacattctgt

SEQ ID NO: 9556 - RNA, 4103 nt, Homo sapiens
  source 1..4103: mol_type = other RNA
agtgcctgctatgtgccaggcatgttgtaggcaattttcatgcatttgttcatgctatttccagtgcatggaatgtcctgcccaaaatctgtttcctggaaaatatccacccatctttcaagtgttggtacatggtttgtataaatttggtcatatctgtctgtctcactttctgttccttcagtcagtcagctttatgcaaatgtcaactgcagaaagtcctaatacaattatgtctactgggccataaactctgaggaacaggtccatgcctcattcatcatttcatccctaacacctgcctagtatctgacacttacattaattcatcttagccccaattagtcctattcttctttcatctgtgacaaagaataaaataagcatgaaaaaacttcatcagacactactaggttatcatttcagaaatcagaatagaaatacataaatataagaaacttgcaggagcataaggatgaatcttaatggatgaagcccagagaattcatgaacttcctcaagttacgagacacattaatggctcagggtttcttcttctttttttttttttttttttttttttttttttgagatggagtctcactttgttgcccaggctggagtgcagtggcgcaatttccactcactgcaagctccgcctcctcggttcacgccattctcctgcctcaacctcatgagtagctgggactacaggcgccggccaccacgcccagctaattttgtatttttagtagagatggggtttcaccgtgttagccaggatggtctcgatctcctgaccttgtgatcctccctccttggcctcccaaagtgctggggttacaggcttgagccaccgcgcccggcctcagggtttcttttataactgtgatcaggaagatgtgcttttctttctacttggttaagcaactaatcaaactcagcacaacaaaacaaagattctccttttctcccaagaagttcaacagttctagcgttgtagaacatttcacaaataaaaccatcctagtttccttttcccataaacagttgaacacatcagtgtgataagatcacctcacactatttcttggcttaatgctagcattgcctcctgcatacagatttctcttacccttctagcagatttaattgcttcttcccctgtattcccacagcactgtatatactctattatagctagtttacgaataataatattaattctggaccataaaattgcaactggtcaatgcctggcatataatgaacactcaaatgaacaaggaattgaatcttgctttaatgaagtaagtcaagactaattatgtcagttccaatcttaagaacgtccttggcttttaatgaggggtcttcatctttgaacacagatttagtttcagacagtggtttttgctgcctgtaataactaaagtttgcaaaaaaattaattatttgaggacactatatttttaagaaatgaatttccttaaactattcctacaagggtaatatacagtaagtgaaaaaccactaacacggtagttctcatagtggttgcttttatgtatgcatacttaagataattttaagtggttagaataggtccagagaacacctatattctatggtgttgccatttaatgttttaattatttaaaatacttaaataatttaatatttaatttgaaaaattaaatactgagtttgttgtgggcaaattagtggtgataaaacattattaatctaaaatctgctcttaaaatttgttcagattatcattgactgattggccccgccctccccatattcactcataatatgatttgttattttgtgattcttgacagttaagaaagcaattttaatacctgaaatgcaagtctagctgtggcttcattttaagaatttggtaattttgtaaaagtgcttgaatgcttgttttaccattgttatatctcaattcttataagaccctcagcagaatcaatttacatgactggcagtactaagccactttaaaattattttaaataattttatttgcttgggttctacttgtttgggttttacatactactgtggcatccttcttttaaggatataaactataattagaaatgatatggaaaaaagtgactagaaaacaaatctgaaggcttttaaaaatttcagagtacattagtaaatgctttaaaagacaacccatccaataacatatatgcaagttaacactacaaattcaatgacataagaaaatagattggacttacttttacattcacctctacagatactctataatgaacacactagtatgatgataataaagcaatcaagaacaatttatctctcagtctgtgtatatgtgactatctacatatttatttcacacacacatgccaaatacccacataacttcaatcctatatccatttacctctcagagtgatttaaagtagccacagtggcacataaaaggaaaaaaataatgaattccaggcttcctagtaagtaaagccaaatcaaattgttcaagtgatactatagtgctatttttacaggaaaacacagatttctataatttctggtcatttacttcatcattaaagtactatttgccaatattggtttcacataatgacaataaaacattcttgacttatatactacatgaaaaaaatagattatgagcttattttttgaccagtcatcaaacatgttttcatttgaataaagaaaattcttccagtttaatatgtttatcaatttgttttttcaatgaaacaaagtaaatttacagtaaagttactggtctcaatataagtcttccaatcttcaaattcagccgaacagtacaaggattacaggagaaaaaaaaacacaattaatctcttgtggctatcattttaggggctggttttctcatattgctgaattctaccacaccctgtcgtatttccaaggtttggatggtgctttaaatctgaactgcctgagaagattcagaaagcctttgttcttgggcttacacagtaagcactttgcgtgattcctaatcacatttttatccagaacacagtgttacgggtcacatttttctcaataatgcttatattgattgatgctctataaatataaacatatttacatacagaatacacacactgacatgggggtatgaagttagccagccatccataggaagaatggaataaaaattgcaggaagggtagtgtatgataccaagcccgtacagactatagacgccaatcccaagactgctgaagcaagaacacttctctgatcacgaataattatcttcacagtctcacaaaacttgtcggactggggactgatcggggtgccatatctgcagtaggtcacgaagtgctcgcagttgttccacagcaggctgtagggggtaaagcccagcagcttttcagccctccgcgccacctcctcgttgagcagtgcctttttctggagggactcgtccaggtgattgaccaggatgttagctccgtaggcgaagtcctccactgtgtccacgcggatgctggccactttgacaataacgcccaggatgagacgcttgttggagaccaccttctgcgtgcgccccatgtcgtctgtcagggccaacaggatgtcgggcatcatgtgggcaacacggttgtctcctaggtagatgccatagtgggtcaggtgggtccggggcacctccagcacgtcgcctcggtggaaagagctggtttcataaaaactgttcctccctttgtcttcgcccgcggcgcccgaactaaagagcgtgaagttggagatgaggagcagcttctccagtagtaaagacaccacctccagcatggggttcttcatcctgcaggccaggtgaggtacggcgcaaagtacggccgctgaggagagaggaaggcaaaggaggacagcgaggcctggcgaccggctcagccaagccacaatggggaatgagacggataaggaaccggtggctgacggcggggacagtgagaccagtgctacaagcagccggagaaggagcgcacctgggggccgtgccgggggcagggccgcgcgcggtgctc

SEQ ID NO: 9557 - RNA, 170 nt, Homo sapiens
  source 1..170: mol_type = other RNA
agtgcctgctatgtgccaggcatttttccaggtgctggagatacatcgataagcaaaacagggtcagcttctgtctctcgggagccatctaagggcaactgccacttagtgccagcccacttctctcccttttttcttttttctttttcccccagggtcttgctgtcacc

SEQ ID NO: 9558 - RNA, 1094 nt, Homo sapiens
  source 1..1094: mol_type = other RNA
agtgcctgctatgtgccaggcatttttctacatgctttacatgtattgagtcatttagtttgatgaggtaggtgctattactaaccctacttttcaggggagagaactggtacagagaggttatgtaatttgttcaaggcactggagctgggaaacccaggcattctggctccggggccagtacattaagctggaggagggaggaatgactgcattaaccattagattggcttagttctttgtgtgtgtttgattcaaagaatgtcttatccttagaaggcactcagaatacaaatatttggagaattaatggatccaaaaccatttcactaaacagacgagcagcattggttaaatacaccagaaacatcttttacgtggattaaagtcaatatgcaaatcttttaggaagattaatacatattttaaggacttagtaacttattacatgtttggagtatctgtaatcgaaagccttaaaagatagtaatagggctgagaatattactccctccccccaaaaaatattttttagcttttcagtttctttaaaaaatttttgttgcttgtaaagaacagtttttcaaagtctacattttttaaagcaaaatgagctttaagccacaagttctgcctcaaatttcattggctttcctctaacatttcattttatgacttgagtttagaatcatagcacctggcatggaaaggcctccagaggtcctccagtacagccagccccaaacagtaatgtcttcggtgtgatctttgtctcgcttttctaggcccacagacaagcccacgaaatgacaggtttacagcctggatttgaagagtcatttcctgtgtgtctgtaatattttggtatgcagggtctggaactcctctttctttcccttgtttaccattttctgtaatcccagcactttgggaggcttaggtgggaggactgcttgagaccaggaattcaagaccagcctgggcaacgtagtgagaccgcatttccaatagggaaattatgaaacagccatgttttaatagcactttccagcccactgccgaaagagctgtggaaatccaatgttagtcttgtt

SEQ ID NO: 9559 - RNA, 76 nt, Homo sapiens
  source 1..76: mol_type = other RNA
agtggcaaagtctttccatatgtatgtatgtatgtctgttacacatatggaaagactttgccactctttaaagtga

SEQ ID NO: 9560 - RNA, 79 nt, Homo sapiens
  source 1..79: mol_type = other RNA
agtggcaaagtctttccatatgtgtaacagacatacatacatacatatggaaagactttgccactcttgaaagtgaaga

SEQ ID NO: 9561 - RNA, 1687 nt, Homo sapiens
  source 1..1687: mol_type = other RNA
agtgggaggccagggcacggcagggggagctgcagggccgtcggagggacctcagcgtctgagccctgtcctcctgtaggaaagttcatcaccctagaacacagccagggggcagtgccaaagatgcggcaactggaggaggacatcatcaggctggcccaggacatggaggagatgaaggtagggtgtgcaacatctctgcaggggtgggggtgggcgtgagggtgggcgccggtagatgcataacagctgagcacccctccctccaggtgaagctgctggagctgctggagaagatgttgcggcttgtggtgactacaacgagggacacagcaaattcccggccactgccctgaagcttgctgatgagcctggtccaggagccccagccccccaggagcttgtgggtgctgataagcatggtggtgagtagagtcctcaggcagggtgggcaggcaggggcaggggaggctctcactgcactcggatccccacctccttctctccaaagatctttgtgaggtgagcctcactgacagcgtggagcacccaggcttgtgcagcaactcccgtatgccattcttttgctgggcttggctgcagctaggcgtcgtccacgggcccccgtagctgtgctgacggtgttcgtgttgatgttgccgatgatgctgagagcctctttcagcacgtggtgcatgcgcagcatctcgtcgcgccgctgtgcctgctccgccgactcctccaggagtgtcttctcgttcccacgcgagtgcaggttggacagcagctctgagaagatgaactccttggtctgcctgctccgccgactcctgcaggagtgtcttcttgtccctacgcgagtgcaggttggacagcagctccgagaagatgaactccttggtctgcctgctctgccgactcctccaggagtgtcttctcgttcccacgcgagtctcgtcgcgccgctgtgcctgctctgccgactcctccaggagtgtctatttcttcccacgcgagtctcgtcgcgccgctgtgcctgctctgccgactcctccacgagtgtcttctggttcccaagcgagtgcaggttggacagcagctctgagaagcagcatctcgtcgcgccgctgtgcctactctgccgactcctccatgagtgtcttctcgttcccacgcgagcgcaggttggacagcagctccgagaagatgaactccttggtccccatgaggcggtgcatgcacattgtagatcatgatatgcatggtggtcttgggcttcgcaccaaccatgaggtcccacacggtcttgttgacaatggccatgtaggagtccaccaggttctgggtggtttccatttgccgctccagctgtgggtccatggagtgcatgaagctgtgggagccattctcctcagccttgctgtccttaccctggggttttacgtttcttgtctcaacactaacatttctcactcctccacaagttgaattgctcactccagccaactgaagcatgctcttcttgacacagttagctctcggcacatggtcggtgcttccacaagaaccaggagccgcagccgcggctcacgctccactgcaacagacggtggggcgcgcggcggcggcctcgcagggcagggcgggggcgcagatgggggagtctcgggaccaacggcagcctaac

SEQ ID NO: 9562 - RNA, 73 nt, Homo sapiens
  source 1..73: mol_type = other RNA
agtggttcttaacagttcaacagttctgtagcgcaattgtgaaatgtttaggaccactagacccggcgggcgc

SEQ ID NO: 9563 - RNA, 28 nt, Homo sapiens
  source 1..28: mol_type = other RNA
agttaggattaggtcgtggaagccacag

SEQ ID NO: 9564 - RNA, 14085 nt, Homo sapiens
  source 1..14085: mol_type = other RNA
agttcttcagtggcaagctttatcaaaatcttccttaaaatgcttcctagaaaccaaattcttctctagttcttgtaaccggtgactgcacttttgtaaaacactgtcatagacactctgcaattcctgaagcttccccagcacttcactcttttcctgctctgtgacttccttcattagttcgcgaccctgggcccaaagtccagtgacttcattttggtaagtcttgaggctggcttgtgcactcttacatgttttgacttgtttgctcacatcatctggtaacagacagatgtgttcacggaacattatctttcgctcatgttgctgaatttggctggtggcctggaacactgccatgagaaactgggttttctcggacaaggctttgtttaagtactttcttcgctggcccactaagtcactgagacaattcacgtggctttgtgcatcagagagagccttctggatgacctgtcgctcattgagaccaagatctgccatgaccctgtctgcgtcctttataagcgatttcaggagcatctgcttggcctccagttcactgcagatggccaggtgatccatgagaaggttctgagccatatctggaggagggctctgcttaagggcctcggcgatgttgggttgttgctcttctgcccactccattagctcctgaaatctggactgcaccacatttaactcctccaagttggtgactgacacttggattttccttttaatgaggtcctcaagctgaaaccaacgttgctctaaatgactcgtctgttctttgactaactccttgtcatctaaattcagatgctctatcattttctgcttttgatctttcagatcttcaatagcatactttctctcctgcaatgccaatgctaactttttcaaagcttccaggtggacagctgtactctctgcatcagatctggccaagttatcccattctgtagtaaatttttctaggaacacttcaacaacattcatacagtcatggtaatctcttgttctctgaagatcctcttccctttgcaagcacaggttgttagactgacggcacaaatcgagccactgatcatttaaatgatttatttccttgtgttcaggcgattcctccttctttgttaacttattcaccttttctattatggtgttcacggatgcctgtttgctctgtagtttcttaacaaaatccttaacttgtgaaaccatgttctgtgcaatgttcagctccagctcagagtgcctcctcttcatgttctgcagttgctgatcagcatcttgcaggtaaatccagagctcagacttcaggtgcttgatctcttcccagccctgagttaagttctgggcctggacaagcttttgttcaatcgtttgctctgtttgttgaatgtcttttgctgtggttttcaccgaagcatttgacaggtcacacatggagcaaaggagatctaggtaggtccttgcctgctcttgcaaagctctgaagtgtttgacctgcttaatggcttctgccctactaagaggtggttgaggacttggctctaaatccggctggactgcagaaagccaggcctggcactgctgcagggtgtcttgtcggctgacgtgcttctgaagttcgtgttccaaactctggtacatcctctgagctgtgctgcagatcgctgagtagctgtcctttgtgccctgcagatgagcatgcacgttttgtttaagtttcgcttgcaggtggtctgcacattggccaatcaaagtatcacctttcatttgaagattgttcaaacggtcttcaaaaccagcaatttcttccatcattgccttgtggtgggccaattgctgggtgattgtctccaggctgcttgtctccaggaggtcaggtgccaccagtctgccagacatctgcagcagccacttttcgacctcttggagctcactgttgtagtcttcatggtctttgactttcgcctccagactgaagacatgctcctttcctatgctgcacaggtcctggtaatcactttgaagttgatctattttgtcctttaaagtgacgtcctgcaccagttccaaaagagcttcacccttctctctcactgactttactgatggttcatgggacagcaccgtttgttgaagtgacttgtatttagataactgagcttttttctcatataattccattttgggttcttcaggaacatgtagaatttcctggtattctgctatccactgtgtcagtgctttgcatttatctgagaattcctttgctaaatgaagacctttttccagcgtcatgtgttctttccggacagtgctggtcagttccttcaactgctccatgtgatcatgaatctcctttcttaacctctctgcctcgccttcctccaagtatttaacagccctctctcctttctcccgggctgatttcagcaaactgtgacctttctccatgtctttgagcaaaacctccaacgtcttcaatttcttccccatcattactgtatctactttgtcaatcttggtagccacattcttgaagtttttatgagtagagccataccaatcagaataggaactgagggatgattctgattcctccaaactctgaatctcctcctccaggaattttatttgttccagcacttggagaagcagggcctggtatctggaagtcagctgggtggcctggcaacccattctgctgttcacgtggctctcgtccagtatctcctgagctctagctcccacttcctcaacttcatctctgtatgcagtcacttcttcgtgccacttcttcatctgatgtaattgtatctccttggttgccctgttagactgacgtctggtcctgggactaactttctcctctgctgttttgagccattcatctacttgctgaaacttttgctccattagcctcaatttgttcaccacgttattgaactgagttcgagtctcggacagcctgtgctggtaagcctgccagtcttgccggagagactctaaagcccggtcctctgcctgtgggatacctgatgggatcacatcctctctggtgtgcagcactgagttcaacagggcctgcccctctgcacagtgtacctgtagctcctgaagatcacgcaatgttgtctcatgagtgtgggcatcaccttcaagaactgaatactggtcgagcttttcttgttcttgccccaaccaaacttcaaatgcctttaggtctctctgatactcttggtgcaggcggacaagtttttcagacttggttacggcttccttggccctctcttggatggctctgtatcgttcctgtagatcctggagttctagctgggtgacatagtgttctgtcatgccagcccctttgacttcgatggtctccagcaagctgctgtaactcagcacttcttcatttaataacttggcttttccgagcatcgttgttttatcccgcagctccgcatgctgcctttctgattcattcaggttggcttccatactatccatccaaccggagaactgtcgaacgccatcctgataacttgtccacttggagagagctccttcgagttggcttttacaacgaatccctgcagacaaaagggatgcccacatatccttcacactctgcagctgctgctgaatagtgggaatgccttctggagaagtattctgaaggacagattctcccctggtcactatcattttcatctgaatctctttttcctgtttgactgataatagagcctcgagcttgagcgtcctgctgtccagcacacttttgtcggatgtcgggtggcagtatgaatccagcatgtgaatcgcatccgtcatccagtcttgtaattctttaatcccaagagagaactgattgtgttctgcaacgattctatccagtcttgacactttctcctggagcttctgctgctccctcctctttgctggcagatcatagaggcgattgctgctttcatggaccatcttctcagttttactcagccagtcctggataggctcagcacttacttcaaagtccttcatttggatctttagattctctagagcagattctttttggtggagatttgaatgaaaatttttccaatcttcttttgcagctgtaactttggcctggatccctttcgctttctctttggtcagcagggtactcagaagttcccctttagacagcatcatgtttagcttgtgctgtccattttcactttctgacaaaaactcctgtattttctgaagactagttgaaacttcacttatattttgaggtatatcaaaacacttggcggtagtgatttttgcattaaccaaccactgctggaaatccctgaaggcctttcgaaatctttgctgtaaaatctgttctttattctggcagcccttggatgcttgcaaacaaagacaattatactctttaatcaagccagaaacttttccactgtaggtactcaggtctctggaaaatcgacaaagttcattcagctgagacttgagatcctctgttctaggctctgctttttgcaaagcatccagtatctcttgtcctttgtgccagcattccactatctcctcatccgtgttcttgccttccaggagggttaactgctgagcccaggttttcagaagggcactgaactgttccagggcctgctccagttgagccacttggcctgagaattcctgctccgaaagggccatctggctgaccaggttctccaaacagctctgcgtttggaatacactgtcttcccactgcttccagtcggcacgcagggcctgcatctccgtgtgcatgagctcacacccactggcagttgtgttctgtttcacttcgggagccagcgactccactctgctgagacggcttgcaccaatctctctggaatctatcagctccttaatttttgataactttttctgggtggctgatgaatctccagacatatctgaccaccggtgaagttcttcctttgctgaatggagccaatctgtgaactcgtggaccgcatctaaatacattagatgatctttcacaatctcttccactttcctcattttttccttggcaacagtcattatatcattaaactgtgttttcagctcctcttgagctgtgtccttgaaagactcatcctctgtcttttcgtagagctccctggacttcgcaattagacggtgaagggctctcgtgtgatcttctgcctcagacaggatggactggaggtggtcaagcaggacgaacttctctttcagacctggctgtggttgtaagggatgttctattttttgatccactgattccatccactgctccaactggtttttcctctctacatagtcattccattggctaatcacagactctaaagtgctttgagcgtggacggaggagctcatgatgtcagcccacacttctttaagggtctctaactgagtctgaatcaccctctgaccttctttgttgctacttctcaaggcctgttcccccttgccaatggccatattcaacttaacttccccttcacctttcatcaggagaatatcctgtatttgtgacagccgtttctccagggtgtctttgctcccaagagtgctctctgcacaggccagtctgtcctgaatggccttcacccagaaccacatgctttgcagtgcttcctccagggcttcgtgctcctgaagggccacctggcagctccggagtttctctttggtcattctaagtaggttctggtggcttgtgaggagctgggaacacaggcggccctcctgcccagcaccgtggccttcttcactcagaagctgccctctctgggaaagcttatcaagagactctcttgcagccagcagttctcccaaaaacatttcaactttatgaacttcatttttcttctcaggaatgtgctgtttactctctcccaagttttccgtattgaacctttcttccatttcatggatccataagttcagttttctgtgctgatcttcaaagcttccaagttctgaagcacagtcttgaagagcctgcttatctttaaggcattgtttcagaaatgcttgaaactcttcattggcctttgtgatttgttcttgaatgctactgacaatttgtttagacaaatgtgcatacaaagtttgtccttcttgagtcactgcatcaagtttgctctgcccatcactgactgagtccaaaatgttctgaagatcatggagctttgcttctagaactttgctgtcaccggtgcgatctgatgattcttttgctgctgcctttgctcccaaaaaccattcttggaattcctgcatagactcactgaagtgtttttccagagattcctgcaggctggcctgggttttggagcacaactggctcacggcttcatgtttctttatcagaccagtcattgcacggcccaggctctccaactcagctgagtggtacttgcggcacaagctattgagattttcttgggtagagctgatgttgctttgttgactttgaagttctttttgtatatccttgacttttttcaatgcttcacaagtctcattttgggcacagttcatcaacgattcttccacttttgtgaaccatgttgttatgtcattaataaacttctccacttgtgtactttgagccgtgaaatccttcagggttccttttgctacttcagttatttctttggcatgctccagtttctgcattaagtctgcttctataaactgaaggtctggcggtgtttctagatttttagttaattctttcagatcattaactttggaatgcagttcttccaatctcaatgctttgtttttaacttcagactcaaattctttaagcagttcttcagctctgaggtggttatccaggttgctgatgttttctgccatctgtggaacgcagttgtttgaccatccctcaatctcatctctagttgacagtacatcatcccaaatggacaggcttactctcagcctatccatgttttcttcaagtttctctgatacatccagccatttgtccacggtgctctccatgtctgttttcaccaagctgaaatcactactgtgaattttcttcagctcagataacaagtgttttcctttgctggtaaagttatccaagtctttctgtttgtaattcattttgttcttggcagtttcatgcttggaaaaagcccatttaagatcctcctgatcttttatggtagttctggttacaatcacactgctggcattttctaagactttagatacagctgatttcaggttctgatattctctcattaagtcaataagtccacagcactgaccctgattttcatgaattagtcttttggtatcatcccaggtgacctctaagcggtttatctccctgtcaacttcaggtgcaaaagctacatctttctgggcaatttgcttggctttgtctttcaaccaacatagttcatgctcgtgagaattcaattcatcttctagctgattaaacactcttaacctctgctgaagagcttggcgggtaggttctttcaatcgctctttgtcagtcctttcttcaatgtcctcaatgcttttcagaagctcctctttctggtcttggaatgcttttttcaacactgccagagcatctgcctcactctgcttggttcccagaaggttctggatcctctctacctctccacagagctgatcagccgtggctctgcaggaagtcctttgctcagagctcccgattttcagatggtattgggctttggaaagaatgccatccagactgacggcagcagattctaatgctttagcattttgaagagcatcattgaggtccttttctatcaaatcagactcgttcttattcatactgttggttgcttccactgtttgcctcagctggcggagaatgccggacagagaggcatggctctggaggaattctgccaaatgggacagggcaagctgccgcctctccacaacctggctggcctcctcaaacagctggaagcagtcctcagcctttccctgcaggaggtggaggtcctcagcacggcccagagaacccaactttgctaagtgaccctgcagactctgcaattcgccctttttgctctctacttctgctgcgtggtccttatgccgagtaagggctacttgatggtccattatgctaatctcagaggtagtttgtaattcactgagaaacagtttaatccagacagaaaaggaaagcagcagctcatcaaattgctggtgttcagcaaccacagactgaagaaaattaatccttttgttaatgatctgtggtaaatctctccatctctcatccaactgctccaaatgtagtttcatcattttcacatcatctttggaggctactgagaacaatgattccttcaattgcaaaagtttgctatagaatgaggcctgggatacaacttcattttgcagtgcctgtattaactgaagttcaccttccactttgactctgtctgcagaaatgtccatttctggggaactggctttagcttcaccccgctctaaccaggtcaaaaaggatgatagttctttctctagcctctgccagtgggccagcagattctccagcgccgtctgtctctccttcgccctccttaggatgtcctcgtattgctgctgtagagccgcagcctcctgaacacaggaatctctgttcacaaccttcctggcactggctgagaaggcagtgatcgcgctgctcagtgactccagggcctggcagagatccatatgttcttgaagaactttgtatgtttctgtagctgaagaacatattttaattggaacagcaagtttatcttcaaattcagacacagattgctggatctttctaaggttctcttcaaacttttgctgctgagataaatgtcccaggattgttccttccagacactgtgcatgctctcgaagctcttccccgtatcttcttatttgtgtcaacttggctttaattcgagcagattctccagtggtaacaaactgagcaaaagactgggcttcttcttctaatcctacaatgctgctgagcttactttctatttcctgaattgtgaccttaatttggctgatttgcatgtccatggcagatgacgaagtttccaaggcattgagttctttttctttctcagttatccagacggacagagtctcaaaattactgccaaaatgatcccacttggttttcaccatttccatggttttaatatcttcttcaagcgtgtcttctaattttttgacttgttctttgattgacttggcctgctgttgaagcagctgcttattttggggcccaagcggtatctctgaagcttcctttacaaggttctcagcctggactgcaatactttctgtccgtttagaaaactcctttgtttgttccagttctgaagataaactttccaaactgctaaaactcaagaagcgttcatgactggaacctgtttgaaaaaggtatcttactactgtttctttgtttgtttcaaatcgctcccattttcttaatgtgacctggatgcggcgttcctgcctctcccggctgcgctccaggccatccagtgtgctctccagcttccgcagctcctcgtggcctcggtcaggcagccccccttctccctgctgcgcctgcgcgatctgctgctgcacatctctcttctttgctgagatccgctttgtcttttgctggtgatgaagaagtaactgctgtgcttcaaacagattttcagtatccaagatcttctcagcttgttcctggacttctttagagccagaaattaattcttcgagagaatttttgactatttctttgtactggacacagtccccaaaattgcttagcatcttttcaacctctgacagcagcgtcacaagagccttgaaagagctggataattttgccagctcatctccctgcttttgggcttcattctcagaagaaacttctgtcaaaactttcagcctggatttcagccagctgagggtctcaccccttttggtaacaccatttctgatctcttcaacggcacgtttaacctctccgtggttggcagtatcgatggcctcacccttgatcccctttaattgtgtctcatttgtagatatccaagatgagaactcagagaatctgctagtgtagtccttccacttgtctgggtcttccatgagcttcctgtaggtgctgtcaatggcagctctgagctctttgagagtcacgtgacaggttccaggtgtgtcccttactgggtcccgcactgggagtttcacacagagttcctcgatgagctgtaaccttttctcacagagatgatgaggacctttgtcactgaagaaaaccctgtgctctttaattatcttttcactgccttcctggggcatcagcttggtctctcgatccagctcagttctgcattcttctacagaggctaagaacctattcttctccacatcaatcttcagatgaagcaaatgataaggggcttctccttgaagatccttccattgtttgtggagctttcgaacagcttcctgcagcccctgctgctcctgctctggaaggatgtcggtgagttcatcacaagctttcaggaaagcattgagcaccctctgatccagctgactgaaaaactcagtgtgtctccgcaggagctcctctggatcccccttttcctccaggccctcctgagcaatccgcagtaccttctccaactctgctcgagactcctcaaacttcttcatcaagcgactgttggtttccacatgcttcttccaatctccagttttctttaccatactctgaaaagcaacatgaatatctgcaatctgtctttgtagcctcgtctgatcaaaatgctttaacacgttgctcaaggtcacaaacttttgaacactttgactgcctttctcaataagtgtcaaggttttcttacagttttcttgacaagctaacagttcctgatgtttttgtttaaaaagggcactcgattgtgcctcacgctcaagaactgtgataatttcattgattttcccaagtgagtcataaaaggacgtcatctgcttttctaattcctccaacggaatcaacagctgctgagactcataaaggagtggggagtaacattctttgaccttggttagctgctctttgagctttgacatggtcgcaaacatttcttttccttcttcttgggggctttctttggtaatgaggtgtgctgtctttgtaattatcttgtattgggcatccatcacaggcaccctctgctcaatatcctccaagtcttgaattaatagcttgacattcataaaagagacttctaagggttcagaaagtttcttatgggcttccgttgcaaaagcagacagggtaacaacacagtctgtgtattccttcttcattctgtccatctcatcagcttgagcatattgcttgacttccataaacaactccctccaccgcccatttagcaacagtaattgctgcttcaggtcacgggaaaccatctcatcacaggtttcaattagaaaattgccagcatcgttcatggcagtatgctgctgaatccaatgaggtaaatttcgaaaaaaatcctttttggcattttctgattgattgagcattttttcagcatcctctagccaggcttgcagactagccactgtattgccatagcgatcccagttagagatcacttcttccagcatgctcctcacactcctcacttctactgagagattcctccactgagcggtggtttcattcatgaatttcatcacattctcagcttcttccactgaaccatctgctttgacatacatctcagctgtctgtttcaagatctggtatgtcacctcatattgttcaaagaacttgctattttctataaaagacacgtagttttgtagaagctgctccactgactctctcctcccgtacttaatgatccaagacttcagctttgactctgcaagaaccagcagtgagagcagacggtactttaattctaaaaattccattttcattaggtgtagctctgatgtggaggaaacaaaatgaaacctctcggccatgtcctctaattgatcaggtggcactggaatcccgttaacagacctggtccggtagatttcatggaatgctcttttgtgggcatccgtgttttgaagcagatccttatgttgctcaagtttccgttgtatcgtgtttgctgtttcctcgtggacctgttgaacggttatttcctctctcagggccacctccgctctgtacagccaggcacctatggtgcccagaggtgcaggaagagatttatcaagctgtatatgccagtcaaagagcctggaggtcactctatcccaagattgttttaccaatgcttggtcaagtgacaatttaccgtctctgtgtaatggttgtattaaatgttcaatctgtttcctcttcatttcatattgaactctgaagtgcttaaatgactgatatttatcctgtaaatttgattccaccatctgtgctcttgtcaaatctctctcaaattgttctatccaaactttcatttccttaaaaattactctgtcttctctcttaaaattttgtacagaatttgcaaaagatgggaaacctggaagtatttcatcatcctcttgcccatcagtgcttgcattgtggatgtcaggataatgtttcagaaactgggctacataggtcataatagatttctcatctggtttatccacatcaacgtcttcaggatctagcagtcttgggatccccagttctgtttcggcgatagtgaaagcatcctccaaattttctcggttggatctgcctttcactgtctccaagtccaccaattccggtcgaatggcatgaataactgaatgaaaggcaaccccgcttctccaactcttcccaaaatcttttacttctattccagtctgcttgccagctgtgtactgaacccactttaataaagccttcttagcatttccttggatcttggtggtcaccttccgtttacttggtgggctgggagtctcagagctaactatgctgtccacggaggatgcgctgctggacaaagactggagctggggcaggttgctggtcaactcttcaatctggaaatatagaataatggtccacatcaatccaagaactattgagggtcggccatcagctatatcggtggagttaatgttgactaatttaatcggtgatcctctgtgcatggactttcttccttcgaggaacttgagtgccgtgccaatgttagccacagcatggattcgcttcatccggcgtccttgttcacaaggcagtttctgcccagacaggacctccagaagggcaagcagtttaacaccatctttcatgtcttcaaaaagatcgtccaccaccattggaggtttccgcttggccagatgagagttgatccattttgtgaaagttcgtttttgtactatctcttgctcatcttgcagcctctgcatcacattggcgatatcccgaggacaccgggaggcccctctggaggttgccatggtccctccggaagcacgaagccaacaccaagagactcttcactggaggcagcacagggctacaccactctagaaaacatgcttggacttttctagatctattctgtcataaatgaattccaggcctttgcagcactcaacaaggaggcagctctcccaaagactgaactgcttctttttcttcttccgttttaagactgtcctcttacatgaactcaagaaccttctctctcggcctcgttcagtttcccagcagcaaggcgaagcgagcgaacgcttcctcccggctctctgcgcccaggctcggcgggaccccggggatgcgcggctgtccgcccgccctgtcgccgggatcgggcgcggtctgcaggactgcgggagcccagccgccctggtgacagaggacaacaatctcagcccgctgcggccggcggccgcggcccggcgcccgcgctcaccctggctggctcgcccacactcact

SEQ ID NO: 9565 - RNA, 11681 nt, Homo sapiens
  source 1..11681: mol_type = other RNA
agttcttcagtggcaagctttatcaaaatcttccttaaaatgcttcctagaaaccaaattcttctctagttcttgtaaccggtgactgcacttttgtaaaacactgtcatagacactctgcaattcctgaagcttccccagcacttcactcttttcctgctctgtgacttccttcattagttcgcgaccctgggcccaaagtccagtgacttcattttggtaagtcttgaggctggcttgtgcactcttacatgttttgacttgtttgctcacatcatctggtaacagacagatgtgttcacggaacattatctttcgctcatgttgctgaatttggctggtggcctggaacactgccatgagaaactgggttttctcggacaaggctttgtttaagtactttcttcgctggcccactaagtcactgagacaattcacgtggctttgtgcatcagagagagccttctggatgacctgtcgctcattgagaccaagatctgccatgaccctgtctgcgtcctttataagcgatttcaggagcatctgcttggcctccagttcactgcagatggccaggtgatccatgagaaggttctgagccatatctggaggagggctctgcttaagggcctcggcgatgttgggttgttgctcttctgcccactccattagctcctgaaatctggactgcaccacatttaactcctccaagttggtgactgacacttggattttccttttaatgaggtcctcaagctgaaaccaacgttgctctaaatgactcgtctgttctttgactaactccttgtcatctaaattcagatgctctatcattttctgcttttgatctttcagatcttcaatagcatactttctctcctgcaatgccaatgctaactttttcaaagcttccaggtggacagctgtactctctgcatcagatctggccaagttatcccattctgtagtaaatttttctaggaacacttcaacaacattcatacagtcatggtaatctcttgttctctgaagatcctcttccctttgcaagcacaggttgttagactgacggcacaaatcgagccactgatcatttaaatgatttatttccttgtgttcaggcgattcctccttctttgttaacttattcaccttttctattatggtgttcacggatgcctgtttgctctgtagtttcttaacaaaatccttaacttgtgaaaccatgttctgtgcaatgttcagctccagctcagagtgcctcctcttcatgttctgcagttgctgatcagcatcttgcaggtaaatccagagctcagacttcaggtgcttgatctcttcccagccctgagttaagttctgggcctggacaagcttttgttcaatcgtttgctctgtttgttgaatgtcttttgctgtggttttcaccgaagcatttgacaggtcacacatggagcaaaggagatctaggtaggtccttgcctgctcttgcaaagctctgaagtgtttgacctgcttaatggcttctgccctactaagaggtggttgaggacttggctctaaatccggctggactgcagaaagccaggcctggcactgctgcagggtgtcttgtcggctgacgtgcttctgaagttcgtgttccaaactctggtacatcctctgagctgtgctgcagatcgctgagtagctgtcctttgtgccctgcagatgagcatgcacgttttgtttaagtttcgcttgcaggtggtctgcacattggccaatcaaagtatcacctttcatttgaagattgttcaaacggtcttcaaaaccagcaatttcttccatcattgccttgtggtgggccaattgctgggtgattgtctccaggctgcttgtctccaggaggtcaggtgccaccagtctgccagacatctgcagcagccacttttcgacctcttggagctcactgttgtagtcttcatggtctttgactttcgcctccagactgaagacatgctcctttcctatgctgcacaggtcctggtaatcactttgaagttgatctattttgtcctttaaagtgacgtcctgcaccagttccaaaagagcttcacccttctctctcactgactttactgatggttcatgggacagcaccgtttgttgaagtgacttgtatttagataactgagcttttttctcatataattccattttgggttcttcaggaacatgtagaatttcctggtattctgctatccactgtgtcagtgctttgcatttatctgagaattcctttgctaaatgaagacctttttccagcgtcatgtgttctttccggacagtgctggtcagttccttcaactgctccatgtgatcatgaatctcctttcttaacctctctgcctcgccttcctccaagtatttaacagccctctctcctttctcccgggctgatttcagcaaactgtgacctttctccatgtctttgagcaaaacctccaacgtcttcaatttcttccccatcattactgtatctactttgtcaatcttggtagccacattcttgaagtttttatgagtagagccataccaatcagaataggaactgagggatgattctgattcctccaaactctgaatctcctcctccaggaattttatttgttccagcacttggagaagcagggcctggtatctggaagtcagctgggtggcctggcaacccattctgctgttcacgtggctctcgtccagtatctcctgagctctagctcccacttcctcaacttcatctctgtatgcagtcacttcttcgtgccacttcttcatctgatgtaattgtatctccttggttgccctgttagactgacgtctggtcctgggactaactttctcctctgctgttttgagccattcatctacttgctgaaacttttgctccattagcctcaatttgttcaccacgttattgaactgagttcgagtctcggacagcctgtgctggtaagcctgccagtcttgccggagagactctaaagcccggtcctctgcctgtgggatacctgatgggatcacatcctctctggtgtgcagcactgagttcaacagggcctgcccctctgcacagtgtacctgtagctcctgaagatcacgcaatgttgtctcatgagtgtgggcatcaccttcaagaactgaatactggtcgagcttttcttgttcttgccccaaccaaacttcaaatgcctttaggtctctctgatactcttggtgcaggcggacaagtttttcagacttggttacggcttccttggccctctcttggatggctctgtatcgttcctgtagatcctggagttctagctgggtgacatagtgttctgtcatgccagcccctttgacttcgatggtctccagcaagctgctgtaactcagcacttcttcatttaataacttggcttttccgagcatcgttgttttatcccgcagctccgcatgctgcctttctgattcattcaggttggcttccatactatccatccaaccggagaactgtcgaacgccatcctgataacttgtccacttggagagagctccttcgagttggcttttacaacgaatccctgcagacaaaagggatgcccacatatccttcacactctgcagctgctgctgaatagtgggaatgccttctggagaagtattctgaaggacagattctcccctggtcactatcattttcatctgaatctctttttcctgtttgactgataatagagcctcgagcttgagcgtcctgctgtccagcacacttttgtcggatgtcgggtggcagtatgaatccagcatgtgaatcgcatccgtcatccagtcttgtaattctttaatcccaagagagaactgattgtgttctgcaacgattctatccagtcttgacactttctcctttgttaaattgcttagcgctagatactgagaagacagctgcgacactctgtgcctaaagctcttgctggcagcttgtccttcccacagctgctgagctttctctttcagcctgttgagctgaggctcgtagcagtgtatttcctcaaggacagactggagcttctgctgctccctcctctttgctggcagatcatagaggcgattgctgctttcatggaccatcttctcagttttactcagccagtcctggataggctcagcacttacttcaaagtccttcatttggatctttagattctctagagcagattctttttggtggagatttgaatgaaaatttttccaatcttcttttgcagctgtaactttggcctggatccctttcgctttctctttggtcagcagggtactcagaagttcccctttagacagcatcatgtttagcttgtgctgtccattttcactttctgacaaaaactcctgtattttctgaagactagttgaaacttcacttatattttgaggtatatcaaaacacttggcggtagtgatttttgcattaaccaaccactgctggaaatccctgaaggcctttcgaaatctttgctgtaaaatctgttctttattctggcagcccttggatgcttgcaaacaaagacaattatactctttaatcaagccagaaacttttccactgtaggtactcaggtctctggaaaatcgacaaagttcattcagctgagacttgagatcctctgttctaggctctgctttttgcaaagcatccagtatctcttgtcctttgtgccagcattccactatctcctcatccgtgttcttgccttccaggagggttaactgctgagcccaggttttcagaagggcactgaactgttccagggcctgctccagttgagccacttggcctgagaattcctgctccgaaagggccatctggctgaccaggttctccaaacagctctgcgtttggaatacactgtcttcccactgcttccagtcggcacgcagggcctgcatctccgtgtgcatgagctcacacccactggcagttgtgttctgtttcacttcgggagccagcgactccactctgctgagacggcttgcaccaatctctctggaatctatcagctccttaatttttgataactttttctgggtggctgatgaatctccagacatatctgaccaccggtgaagttcttcctttgctgaatggagccaatctgtgaactcgtggaccgcatctaaatacattagatgatctttcacaatctcttccactttcctcattttttccttggcaacagtcattatatcattaaactgtgttttcagctcctcttgagctgtgtccttgaaagactcatcctctgtcttttcgtagagctccctggacttcgcaattagacggtgaagggctctcgtgtgatcttctgcctcagacaggatggactggaggtggtcaagcaggacgaacttctctttcagacctggctgtggttgtaagggatgttctattttttgatccactgattccatccactgctccaactggtttttcctctctacatagtcattccattggctaatcacagactctaaagtgctttgagcgtggacggaggagctcatgatgtcagcccacacttctttaagggtctctaactgagtctgaatcaccctctgaccttctttgttgctacttctcaaggcctgttcccccttgccaatggccatattcaacttaacttccccttcacctttcatcaggagaatatcctgtatttgtgacagccgtttctccagggtgtctttgctcccaagagtgctctctgcacaggccagtctgtcctgaatggccttcacccagaaccacatgctttgcagtgcttcctccagggcttcgtgctcctgaagggccacctggcagctccggagtttctctttggtcattctaagtaggttctggtggcttgtgaggagctgggaacacaggcggccctcctgcccagcaccgtggccttcttcactcagaagctgccctctctgggaaagcttatcaagagactctcttgcagccagcagttctcccaaaaacatttcaactttatgaacttcatttttcttctcaggaatgtgctgtttactctctcccaagttttccgtattgaacctttcttccatttcatggatccataagttcagttttctgtgctgatcttcaaagcttccaagttctgaagcacagtcttgaagagcctgcttatctttaaggcattgtttcagaaatgcttgaaactcttcattggcctttgtgatttgttcttgaatgctactgacaatttgtttagacaaatgtgcatacaaagtttgtccttcttgagtcactgcatcaagtttgctctgcccatcactgactgagtccaaaatgttctgaagatcatggagctttgcttctagaactttgctgtcaccggtgcgatctgatgattcttttgctgctgcctttgctcccaaaaaccattcttggaattcctgcatagactcactgaagtgtttttccagagattcctgcaggctggcctgggttttggagcacaactggctcacggcttcatgtttctttatcagaccagtcattgcacggcccaggctctccaactcagctgagtggtacttgcggcacaagctattgagattttcttgggtagagctgatgttgctttgttgactttgaagttctttttgtatatccttgacttttttcaatgcttcacaagtctcattttgggcacagttcatcaacgattcttccacttttgtgaaccatgttgttatgtcattaataaacttctccacttgtgtactttgagccgtgaaatccttcagggttccttttgctacttcagttatttctttggcatgctccagtttctgcattaagtctgcttctataaactgaaggtctggcggtgtttctagatttttagttaattctttcagatcattaactttggaatgcagttcttccaatctcaatgctttgtttttaacttcagactcaaattctttaagcagttcttcagctctgaggtggttatccaggttgctgatgttttctgccatctgtggaacgcagttgtttgaccatccctcaatctcatctctagttgacagtacatcatcccaaatggacaggcttactctcagcctatccatgttttcttcaagtttctctgatacatccagccatttgtccacggtgctctccatgtctgttttcaccaagctgaaatcactactgtgaattttcttcagctcagataacaagtgttttcctttgctggtaaagttatccaagtctttctgtttgtaattcattttgttcttggcagtttcatgcttggaaaaagcccatttaagatcctcctgatcttttatggtagttctggttacaatcacactgctggcattttctaagactttagatacagctgatttcaggttctgatattctctcattaagtcaataagtccacagcactgaccctgattttcatgaattagtcttttggtatcatcccaggtgacctctaagcggtttatctccctgtcaacttcaggtgcaaaagctacatctttctgggcaatttgcttggctttgtctttcaaccaacatagttcatgctcgtgagaattcaattcatcttctagctgattaaacactcttaacctctgctgaagagcttggcgggtaggttctttcaatcgctctttgtcagtcctttcttcaatgtcctcaatgcttttcagaagctcctctttctggtcttggaatgcttttttcaacactgccagagcatctgcctcactctgcttggttcccagaaggttctggatcctctctacctctccacagagctgatcagccgtggctctgcaggaagtcctttgctcagagctcccgattttcagatggtattgggctttggaaagaatgccatccagactgacggcagcagattctaatgctttagcattttgaagagcatcattgaggtccttttctatcaaatcagactcgttcttattcatactgttggttgcttccactgtttgcctcagctggcggagaatgccggacagagaggcatggctctggaggaattctgccaaatgggacagggcaagctgccgcctctccacaacctggctggcctcctcaaacagctggaagcagtcctcagcctttccctgcaggaggtggaggtcctcagcacggcccagagaacccaactttgctaagtgaccctgcagactctgcaattcgccctttttgctctctacttctgctgcgtggtccttatgccgagtaagggctacttgatggtccattatgctaatctcagaggtagtttgtaattcactgagaaacagtttaatccagacagaaaaggaaagcagcagctcatcaaattgctggtgttcagcaaccacagactgaagaaaattaatccttttgttaatgatctgtggtaaatctctccatctctcatccaactgctccaaatgtagtttcatcattttcacatcatctttggaggctactgagaacaatgattccttcaattgcaaaagtttgctatagaatgaggcctgggatacaacttcattttgcagtgcctgtattaactgaagttcaccttccactttgactctgtctgcagaaatgtccatttctggggaactggctttagcttcaccccgctctaaccaggtcaaaaaggatgatagttctttctctagcctctgccagtgggccagcagattctccagcgccgtctgtctctccttcgccctccttaggatgtcctcgtattgctgctgtagagccgcagcctcctgaacacaggaatctctgttcacaaccttcctggcactggctgagaaggcagtgatcgcgctgctcagtgactccagggcctggcagagatccatatgttcttgaagaactttgtatgtttctgtagctgaagaacatattttaattggaacagcaagtttatcttcaaattcagacacagattgctggatctttctaaggttctcttcaaacttttgctgctgagataaatgtcccaggattgttccttccagacactgtgcatgctctcgaagctcttccccgtatcttcttatttgtgtcaacttggctttaattcgagcagattctccagtggtaacaaactgagcaaaagactgggcttcttcttctaatcctacaatgctgctgagcttactttctatttcctgaattgtgaccttaatttggctgatttgcatgtccatggcagatgacgaagtttccaaggcattgagttctttttctttctcagttatccagacggacagagtctcaaaattactgccaaaatgatcccacttggttttcaccatttccatggttttaatatcttcttcaagcgtgtcttctaattttttgacttgttctttgattgacttggcctgctgttgaagcagctgcttattttggggcccaagcggtatctctgaagcttcctttacaaggttctcagcctggactgcaatactttctgtccgtttagaaaactcctttgtttgttccagttctgaagataaactttccaaactgctaaaactcaagaagcgttcatgactggaacctgtttgaaaaaggtatcttactactgtttctttgtttgtttcaaatcgctcccattttcttaatgtgacctggatgcggcgttcctgcctctcccggctgcgctccaggccatccagtgtgctctccagcttccgcagctcctcgtggcctcggtcaggcagccccccttctccctgctgcgcctgcgcgatctgctgctgcacatctctcttctttgctgagatccgctttgtcttttgctggtgatgaagaagtaactgctgtgcttcaaacagattttcagtatccaagatcttctcagcttgttcctggacttctttagagccagaaattaattcttcgagagaatttttgactatttctttgtactggacacagtccccaaaattgcttagcatcttttcaacctctgacagcagcgtcacaagagccttgaaagagctggataattttgccagctcatctccctgcttttgggcttcattctcagaagaaacttctgtcaaaactttcagcctggatttcagccagctgagggtctcaccccttttggtaacaccatttctgatctcttcaacggcacgtttaacctctccgtggttggcagtatcgatggcctcacccttgatcccctttaattgtgtctcatttgtagatatccaagatgagaactcagagaatctgctagtgtagtccttccacttgtctgggtcttccatgagcttcctgtaggtgctgtcaatggcagctctgagctctttgagagtcacgtgacaggttccaggtgtgtcccttactgggtcccgcactgggagtttcacacagagttcctcgatgagctgtaaccttttctcacagagatgatgaggacctttgtcactgaagaaaaccctgtgctctttaattatcttttcactgccttcctggggcatcagcttggtctctcgatccagctcagttctgcattcttctacagaggctaagaacctattcttctccacatcaatcttcagatgaagcaaatgataaggggcttctccttgaagatccttccattgtttgtggagctttcgaacagcttcctgcagcccctgctgctcctgctctggaaggatgtcggtgagttcatcacaagctttcaggaaagcattgagcaccctctgatccagctgactgaaaaactcagtgtgtctccgcaggagctcctctggatcccccttttcctccaggccctcctgagcaatccgcagtaccttctccaactctgctcgagactcctcaaacttcttcatcaagcgactgttggtttccacatgcttcttccaatctccagttttctttaccatactctgaaaagcaacatgaatatctgcaatctgtctttgtagcctcgtctgatcaaaatgctttaacacgttgctcaaggtcacaaacttttgaacactttgactgcctttctcaataagtgtcaaggttttcttacagttttcttgacaagctaacagttcctgatgtttttgtttaaaaagggcactcgattgtgcctcacgctcaagaactgtgataatttcattgattttcccaagtgagtcataaaaggacgtcatctgcttttctaattcctccaacggaatcaacagctgctgagactcataaaggagtggggagtaacattctttgaccttggttagctgctctttgagctttgacatggtcgcaaacatttcttttccttcttcttgggggctttctttggtaatgaggtgtgctgtctttgtaattatcttgtattgggcatccatcacaggcaccctctgctcaatatcactaaactttcgacgattccagtttttgcttcccttcattactccaagtcttgaattaatagcttgacattcataaaagagacttctaagggttcagaaagtttcttatgggcttccgttgcaaaagcagacagggtaacaacacagtctgtgtattccttcttcattctgtccatctcatcagcttgagcata

SEQ ID NO: 9566 - RNA, 14072 nt, Homo sapiens
  source 1..14072: mol_type = other RNA
agttcttcagtggcaagctttatcaaaatcttccttaaaatgcttcctagaaaccaaattcttctctagttcttgtaaccggtgactgcacttttgtaaaacactgtcatagacactctgcaattcctgaagcttccccagcacttcactcttttcctgctctgtgacttccttcattagttcgcgaccctgggcccaaagtccagtgacttcattttggtaagtcttgaggctggcttgtgcactcttacatgttttgacttgtttgctcacatcatctggtaacagacagatgtgttcacggaacattatctttcgctcatgttgctgaatttggctggtggcctggaacactgccatgagaaactgggttttctcggacaaggctttgtttaagtactttcttcgctggcccactaagtcactgagacaattcacgtggctttgtgcatcagagagagccttctggatgacctgtcgctcattgagaccaagatctgccatgaccctgtctgcgtcctttataagcgatttcaggagcatctgcttggcctccagttcactgcagatggccaggtgatccatgagaaggttctgagccatatctggaggagggctctgcttaagggcctcggcgatgttgggttgttgctcttctgcccactccattagctcctgaaatctggactgcaccacatttaactcctccaagttggtgactgacacttggattttccttttaatgaggtcctcaagctgaaaccaacgttgctctaaatgactcgtctgttctttgactaactccttgtcatctaaattcagatgctctatcattttctgcttttgatctttcagatcttcaatagcatactttctctcctgcaatgccaatgctaactttttcaaagcttccaggtggacagctgtactctctgcatcagatctggccaagttatcccattctgtagtaaatttttctaggaacacttcaacaacattcatacagtcatggtaatctcttgttctctgaagatcctcttccctttgcaagcacaggttgttagactgacggcacaaatcgagccactgatcatttaaatgatttatttccttgtgttcaggcgattcctccttctttgttaacttattcaccttttctattatggtgttcacggatgcctgtttgctctgtagtttcttaacaaaatccttaacttgtgaaaccatgttctgtgcaatgttcagctccagctcagagtgcctcctcttcatgttctgcagttgctgatcagcatcttgcaggtaaatccagagctcagacttcaggtgcttgatctcttcccagccctgagttaagttctgggcctggacaagcttttgttcaatcgtttgctctgtttgttgaatgtcttttgctgtggttttcaccgaagcatttgacaggtcacacatggagcaaaggagatctaggtaggtccttgcctgctcttgcaaagctctgaagtgtttgacctgcttaatggcttctgccctactaagaggtggttgaggacttggctctaaatccggctggactgcagaaagccaggcctggcactgctgcagggtgtcttgtcggctgacgtgcttctgaagttcgtgttccaaactctggtacatcctctgagctgtgctgcagatcgctgagtagctgtcctttgtgccctgcagatgagcatgcacgttttgtttaagtttcgcttgcaggtggtctgcacattggccaatcaaagtatcacctttcatttgaagattgttcaaacggtcttcaaaaccagcaatttcttccatcattgccttgtggtgggccaattgctgggtgattgtctccaggctgcttgtctccaggaggtcaggtgccaccagtctgccagacatctgcagcagccacttttcgacctcttggagctcactgttgtagtcttcatggtctttgactttcgcctccagactgaagacatgctcctttcctatgctgcacaggtcctggtaatcactttgaagttgatctattttgtcctttaaagtgacgtcctgcaccagttccaaaagagcttcacccttctctctcactgactttactgatggttcatgggacagcaccgtttgttgaagtgacttgtatttagataactgagcttttttctcatataattccattttgggttcttcaggaacatgtagaatttcctggtattctgctatccactgtgtcagtgctttgcatttatctgagaattcctttgctaaatgaagacctttttccagcgtcatgtgttctttccggacagtgctggtcagttccttcaactgctccatgtgatcatgaatctcctttcttaacctctctgcctcgccttcctccaagtatttaacagccctctctcctttctcccgggctgatttcagcaaactgtgacctttctccatgtctttgagcaaaacctccaacgtcttcaatttcttccccatcattactgtatctactttgtcaatcttggtagccacattcttgaagtttttatgagtagagccataccaatcagaataggaactgagggatgattctgattcctccaaactctgaatctcctcctccaggaattttatttgttccagcacttggagaagcagggcctggtatctggaagtcagctgggtggcctggcaacccattctgctgttcacgtggctctcgtccagtatctcctgagctctagctcccacttcctcaacttcatctctgtatgcagtcacttcttcgtgccacttcttcatctgatgtaattgtatctccttggttgccctgttagactgacgtctggtcctgggactaactttctcctctgctgttttgagccattcatctacttgctgaaacttttgctccattagcctcaatttgttcaccacgttattgaactgagttcgagtctcggacagcctgtgctggtaagcctgccagtcttgccggagagactctaaagcccggtcctctgcctgtgggatacctgatgggatcacatcctctctggtgtgcagcactgagttcaacagggcctgcccctctgcacagtgtacctgtagctcctgaagatcacgcaatgttgtctcatgagtgtgggcatcaccttcaagaactgaatactggtcgagcttttcttgttcttgccccaaccaaacttcaaatgcctttaggtctctctgatactcttggtgcaggcggacaagtttttcagacttggttacggcttccttggccctctcttggatggctctgtatcgttcctgtagatcctggagttctagctgggtgacatagtgttctgtcatgccagcccctttgacttcgatggtctccagcaagctgctgtaactcagcacttcttcatttaataacttggcttttccgagcatcgttgttttatcccgcagctccgcatgctgcctttctgattcattcaggttggcttccatactatccatccaaccggagaactgtcgaacgccatcctgataacttgtccacttggagagagctccttcgagttggcttttacaacgaatccctgcagacaaaagggatgcccacatatccttcacactctgcagctgctgctgaatagtgggaatgccttctggagaagtattctgaaggacagattctcccctggtcactatcattttcatctgaatctctttttcctgtttgactgataatagagcctcgagcttgagcgtcctgctgtccagcacacttttgtcggatgtcgggtggcagtatgaatccagcatgtgaatcgcatccgtcatccagtcttgtaattctttaatcccaagagagaactgattgtgttctgcaacgattctatccagtcttgacactttctcctttgttaaattgcttagcgctagatactgagaagacagctgcgacactctgtgcctaaagctcttgctggcagcttgtccttcccacagctgctgagctttctctttcagcctgttgagctgaggctcgtagcagtgtatttcctcaaggacagactggagcttctgctgctccctcctctttgctggcagatcatagaggcgattgctgctttcatggaccatcttctcagttttactcagccagtcctggataggctcagcacttacttcaaagtccttcatttggatctttagattctctagagcagattctttttggtggagatttgaatgaaaatttttccaatcttcttttgcagctgtaactttggcctggatccctttcgctttctctttggtcagcagggtactcagaagttcccctttagacagcatcatgtttagcttgtgctgtccattttcactttctgacaaaaactcctgtattttctgaagactagttgaaacttcacttatattttgaggtatatcaaaacacttggcggtagtgatttttgcattaaccaaccactgctggaaatccctgaaggcctttcgaaatctttgctgtaaaatctgttctttattctggcagcccttggatgcttgcaaacaaagacaattatactctttaatcaagccagaaacttttccactgtaggtactcaggtctctggaaaatcgacaaagttcattcagctgagacttgagatcctctgttctaggctctgctttttgcaaagcatccagtatctcttgtcctttgtgccagcattccactatctcctcatccgtgttcttgccttccaggagggttaactgctgagcccaggttttcagaagggcactgaactgttccagggcctgctccagttgagccacttggcctgagaattcctgctccgaaagggccatctggctgaccaggttctccaaacagctctgcgtttggaatacactgtcttcccactgcttccagtcggcacgcagggcctgcatctccgtgtgcatgagctcacacccactggcagttgtgttctgtttcacttcgggagccagcgactccactctgctgagacggcttgcaccaatctctctggaatctatcagctccttaatttttgataactttttctgggtggctgatgaatctccagacatatctgaccaccggtgaagttcttcctttgctgaatggagccaatctgtgaactcgtggaccgcatctaaatacattagatgatctttcacaatctcttccactttcctcattttttccttggcaacagtcattatatcattaaactgtgttttcagctcctcttgagctgtgtccttgaaagactcatcctctgtcttttcgtagagctccctggacttcgcaattagacggtgaagggctctcgtgtgatcttctgcctcagacaggatggactggaggtggtcaagcaggacgaacttctctttcagacctggctgtggttgtaagggatgttctattttttgatccactgattccatccactgctccaactggtttttcctctctacatagtcattccattggctaatcacagactctaaagtgctttgagcgtggacggaggagctcatgatgtcagcccacacttctttaagggtctctaactgagtctgaatcaccctctgaccttctttgttgctacttctcaaggcctgttcccccttgccaatggccatattcaacttaacttccccttcacctttcatcaggagaatatcctgtatttgtgacagccgtttctccagggtgtctttgctcccaagagtgctctctgcacaggccagtctgtcctgaatggccttcacccagaaccacatgctttgcagtgcttcctccagggcttcgtgctcctgaagggccacctggcagctccggagtttctctttggtcattctaagtaggttctggtggcttgtgaggagctgggaacacaggcggccctcctgcccagcaccgtggccttcttcactcagaagctgccctctctgggaaagcttatcaagagactctcttgcagccagcagttctcccaaaaacatttcaactttatgaacttcatttttcttctcaggaatgtgctgtttactctctcccaagttttccgtattgaacctttcttccatttcatggatccataagttcagttttctgtgctgatcttcaaagcttccaagttctgaagcacagtcttgaagagcctgcttatctttaaggcattgtttcagaaatgcttgaaactcttcattggcctttgtgatttgttcttgaatgctactgacaatttgtttagacaaatgtgcatacaaagtttgtccttcttgagtcactgcatcaagtttgctctgcccatcactgactgagtccaaaatgttctgaagatcatggagctttgcttctagaactttgctgtcaccggtgcgatctgatgattcttttgctgctgcctttgctcccaaaaaccattcttggaattcctgcatagactcactgaagtgtttttccagagattcctgcaggctggcctgggttttggagcacaactggctcacggcttcatgtttctttatcagaccagtcattgcacggcccaggctctccaactcagctgagtggtacttgcggcacaagctattgagattttcttgggtagagctgatgttgctttgttgactttgaagttctttttgtatatccttgacttttttcaatgcttcacaagtctcattttgggcacagttcatcaacgattcttccacttttgtgaaccatgttgttatgtcattaataaacttctccacttgtgtactttgagccgtgaaatccttcagggttccttttgctacttcagttatttctttggcatgctccagtttctgcattaagtctgcttctataaactgaaggtctggcggtgtttctagatttttagttaattctttcagatcattaactttggaatgcagttcttccaatctcaatgctttgtttttaacttcagactcaaattctttaagcagttcttcagctctgaggtggttatccaggttgctgatgttttctgccatctgtggaacgcagttgtttgaccatccctcaatctcatctctagttgacagtacatcatcccaaatggacaggcttactctcagcctatccatgttttcttcaagtttctctgatacatccagccatttgtccacggtgctctccatgtctgttttcaccaagctgaaatcactactgtgaattttcttcagctcagataacaagtgttttcctttgctggtaaagttatccaagtctttctgtttgtaattcattttgttcttggcagtttcatgcttggaaaaagcccatttaagatcctcctgatcttttatggtagttctggttacaatcacactgctggcattttctaagactttagatacagctgatttcaggttctgatattctctcattaagtcaataagtccacagcactgaccctgattttcatgaattagtcttttggtatcatcccaggtgacctctaagcggtttatctccctgtcaacttcaggtgcaaaagctacatctttctgggcaatttgcttggctttgtctttcaaccaacatagttcatgctcgtgagaattcaattcatcttctagctgattaaacactcttaacctctgctgaagagcttggcgggtaggttctttcaatcgctctttgtcagtcctttcttcaatgtcctcaatgcttttcagaagctcctctttctggtcttggaatgcttttttcaacactgccagagcatctgcctcactctgcttggttcccagaaggttctggatcctctctacctctccacagagctgatcagccgtggctctgcaggaagtcctttgctcagagctcccgattttcagatggtattgggctttggaaagaatgccatccagactgacggcagcagattctaatgctttagcattttgaagagcatcattgaggtccttttctatcaaatcagactcgttcttattcatactgttggttgcttccactgtttgcctcagctggcggagaatgccggacagagaggcatggctctggaggaattctgccaaatgggacagggcaagctgccgcctctccacaacctggctggcctcctcaaacagctggaagcagtcctcagcctttccctgcaggaggtggaggtcctcagcacggcccagagaacccaactttgctaagtgaccctgcagactctgcaattcgccctttttgctctctacttctgctgcgtggtccttatgccgagtaagggctacttgatggtccattatgctaatctcagaggtagtttgtaattcactgagaaacagtttaatccagacagaaaaggaaagcagcagctcatcaaattgctggtgttcagcaaccacagactgaagaaaattaatccttttgttaatgatctgtggtaaatctctccatctctcatccaactgctccaaatgtagtttcatcattttcacatcatctttggaggctactgagaacaatgattccttcaattgcaaaagtttgctatagaatgaggcctgggatacaacttcattttgcagtgcctgtattaactgaagttcaccttccactttgactctgtctgcagaaatgtccatttctggggaactggctttagcttcaccccgctctaaccaggtcaaaaaggatgatagttctttctctagcctctgccagtgggccagcagattctccagcgccgtctgtctctccttcgccctccttaggatgtcctcgtattgctgctgtagagccgcagcctcctgaacacaggaatctctgttcacaaccttcctggcactggctgagaaggcagtgatcgcgctgctcagtgactccagggcctggcagagatccatatgttcttgaagaactttgtatgtttctgtagctgaagaacatattttaattggaacagcaagtttatcttcaaattcagacacagattgctggatctttctaaggttctcttcaaacttttgctgctgagataaatgtcccaggattgttccttccagacactgtgcatgctctcgaagctcttccccgtatcttcttatttgtgtcaacttggctttaattcgagcagattctccagtggtaacaaactgagcaaaagactgggcttcttcttctaatcctacaatgctgctgagcttactttctatttcctgaattgtgaccttaatttggctgatttgcatgtccatggcagatgacgaagtttccaaggcattgagttctttttctttctcagttatccagacggacagagtctcaaaattactgccaaaatgatcccacttggttttcaccatttccatggttttaatatcttcttcaagcgtgtcttctaattttttgacttgttctttgattgacttggcctgctgttgaagcagctgcttattttggggcccaagcggtatctctgaagcttcctttacaaggttctcagcctggactgcaatactttctgtccgtttagaaaactcctttgtttgttccagttctgaagataaactttccaaactgctaaaactcaagaagcgttcatgactggaacctgtttgaaaaaggtatcttactactgtttctttgtttgtttcaaatcgctcccattttcttaatgtgacctggatgcggcgttcctgcctctcccggctgcgctccaggccatccagtgtgctctccagcttccgcagctcctcgtggcctcggtcaggcagccccccttctccctgctgcgcctgcgcgatctgctgctgcacatctctcttctttgctgagatccgctttgtcttttgctggtgatgaagaagtaactgctgtgcttcaaacagattttcagtatccaagatcttctcagcttgttcctggacttctttagagccagaaattaattcttcgagagaatttttgactatttctttgtactggacacagtccccaaaattgcttagcatcttttcaacctctgacagcagcgtcacaagagccttgaaagagctggataattttgccagctcatctccctgcttttgggcttcattctcagaagaaacttctgtcaaaactttcagcctggatttcagccagctgagggtctcaccccttttggtaacaccatttctgatctcttcaacggcacgtttaacctctccgtggttggcagtatcgatggcctcacccttgatcccctttaattgtgtctcatttgtagatatccaagatgagaactcagagaatctgctagtgtagtccttccacttgtctgggtcttccatgagcttcctgtaggtgctgtcaatggcagctctgagctctttgagagtcacgtgacaggttccaggtgtgtcccttactgggtcccgcactgggagtttcacacagagttcctcgatgagctgtaaccttttctcacagagatgatgaggacctttgtcactgaagaaaaccctgtgctctttaattatcttttcactgccttcctggggcatcagcttggtctctcgatccagctcagttctgcattcttctacagaggctaagaacctattcttctccacatcaatcttcagatgaagcaaatgataaggggcttctccttgaagatccttccattgtttgtggagctttcgaacagcttcctgcagcccctgctgctcctgctctggaaggatgtcggtgagttcatcacaagctttcaggaaagcattgagcaccctctgatccagctgactgaaaaactcagtgtgtctccgcaggagctcctctggatcccccttttcctccaggccctcctgagcaatccgcagtaccttctccaactctgctcgagactcctcaaacttcttcatcaagcgactgttggtttccacatgcttcttccaatctccagttttctttaccatactctgaaaagcaacatgaatatctgcaatctgtctttgtagcctcgtctgatcaaaatgctttaacacgttgctcaaggtcacaaacttttgaacactttgactgcctttctcaataagtgtcaaggttttcttacagttttcttgacaagctaacagttcctgatgtttttgtttaaaaagggcactcgattgtgcctcacgctcaagaactgtgataatttcattgattttcccaagtgagtcataaaaggacgtcatctgcttttctaattcctccaacggaatcaacagctgctgagactcataaaggagtggggagtaacattctttgaccttggttagctgctctttgagctttgacatggtcgcaaacatttcttttccttcttcttgggggctttctttggtaatgaggtgtgctgtctttgtaattatcttgtattgggcatccatcacaggcaccctctgctcaatatcctccaagtcttgaattaatagcttgacattcataaaagagacttctaagggttcagaaagtttcttatgggcttccgttgcaaaagcagacagggtaacaacacagtctgtgtattccttcttcattctgtccatctcatcagcttgagcatactttttggcattttctgattgattgagcattttttcagcatcctctagccaggcttgcagactagccactgtattgccatagcgatcccagttagagatcacttcttccagcatgctcctcacactcctcacttctactgagagattcctccactgagcggtggtttcattcatgaatttcatcacattctcagcttcttccactgaaccatctgctttgacatacatctcagctgtctgtttcaagatctggtatgtcacctcatattgttcaaagaacttgctattttctataaaagacacgtagttttgtagaagctgctccactgactctctcctcccgtacttaatgatccaagacttcagctttgactctgcaagaaccagcagtgagagcagacggtactttaattctaaaaattccattttcattaggtgtagctctgatgtggaggaaacaaaatgaaacctctcggccatgtcctctaattgatcaggtggcactggaatcccgttaacagacctggtccggtagatttcatggaatgctcttttgtgggcatccgtgttttgaagcagatccttatgttgctcaagtttccgttgtatcgtgtttgctgtttcctcgtggacctgttgaacggttatttcctctctcagggccacctccgctctgtacagccaggcacctatggtgcccagaggtgcaggaagagatttatcaagctgtatatgccagtcaaagagcctggaggtcactctatcccaagattgttttaccaatgcttggtcaagtgacaatttaccgtctctgtgtaatggttgtattaaatgttcaatctgtttcctcttcatttcatattgaactctgaagtgcttaaatgactgatatttatcctgtaaatttgattccaccatctgtgctcttgtcaaatctctctcaaattgttctatccaaactttcatttccttaaaaattactctgtcttctctcttaaaattttgtacagaatttgcaaaagatgggaaacctggaagtatttcatcatcctcttgcccatcagtgcttgcattgtggatgtcaggataatgtttcagaaactgggctacataggtcataatagatttctcatctggtttatccacatcaacgtcttcaggatctagcagtcttgggatccccagttctgtttcggcgatagtgaaagcatcctccaaattttctcggttggatctgcctttcactgtctccaagtccaccaattccggtcgaatggcatgaataactgaatgaaaggcaaccccgcttctccaactcttcccaaaatcttttacttctattccagtctgcttgccagctgtgtactgaacccactttaataaagccttcttagcatttccttggatcttggtggtcaccttccgtttacttggtgggctgggagtctcagagctaactatgctgtccacggaggatgcgctgctggacaaagactggagctggggcaggttgctggtcaactcttcaatctggaaatatagaataatggtccacatcaatccaagaactattgagggtcggccatcagctatatcggtggagttaatgttgactaatttaatcggtgatcctctgtgcatggactttcttccttcgaggaacttgagtgccgtgccaatgttagccacagcatggattcgcttcatccggcgtccttgttcacaaggcagtttctgcccagacaggacctccagaagggcaagcagtttaacaccatctttcatgtcttcaaaaagatcgtccaccaccattggaggtttccgcttggccagatgagagttgatccattttgtgaaagttcgtttttgtactatctcttgctcatcttgcagcctctgcatcacattggcgatatcccgaggacaccgggaggcccctctggaggttgccatggtccctccggaagcacgaagccaacaccaagagactcttcactggaggcagcacagggctacaccactctagaaaacatgcttggacttttctagatctattctgtcataaatgaattccaggcctttgcagcactcaacaaggaggcagctctcccaaagactgaactgcttctttttcttcttccgttttaagactgtcctcttacatgaactcaagaaccttctctctcggcctcgttcagtttcccagcagcaaggcgaagcgagcgaacgcttcctcccggctctctgcgcccaggctcggcgggaccccggggatgcgcggctgtccgcccgccctgtcgccgggatcgggcgcggtctgcaggactgcgggagcccagccgccctggtgacagaggacaacaatctcagcccgctgcggccggcggccgcggcccggcgcccgcgctcaccctggctggctcgcccacact

SEQ ID NO: 9567 - RNA, 14186 nt, Homo sapiens
  source 1..14186: mol_type = other RNA
agttcttcagtggcaagctttatcaaaatcttccttaaaatgcttcctagaaaccaaattcttctctagttcttgtaaccggtgactgcacttttgtaaaacactgtcatagacactctgcaattcctgaagcttccccagcacttcactcttttcctgctctgtgacttccttcattagttcgcgaccctgggcccaaagtccagtgacttcattttggtaagtcttgaggctggcttgtgcactcttacatgttttgacttgtttgctcacatcatctggtaacagacagatgtgttcacggaacattatctttcgctcatgttgctgaatttggctggtggcctggaacactgccatgagaaactgggttttctcggacaaggctttgtttaagtactttcttcgctggcccactaagtcactgagacaattcacgtggctttgtgcatcagagagagccttctggatgacctgtcgctcattgagaccaagatctgccatgaccctgtctgcgtcctttataagcgatttcaggagcatctgcttggcctccagttcactgcagatggccaggtgatccatgagaaggttctgagccatatctggaggagggctctgcttaagggcctcggcgatgttgggttgttgctcttctgcccactccattagctcctgaaatctggactgcaccacatttaactcctccaagttggtgactgacacttggattttccttttaatgaggtcctcaagctgaaaccaacgttgctctaaatgactcgtctgttctttgactaactccttgtcatctaaattcagatgctctatcattttctgcttttgatctttcagatcttcaatagcatactttctctcctgcaatgccaatgctaactttttcaaagcttccaggtggacagctgtactctctgcatcagatctggccaagttatcccattctgtagtaaatttttctaggaacacttcaacaacattcatacagtcatggtaatctcttgttctctgaagatcctcttccctttgcaagcacaggttgttagactgacggcacaaatcgagccactgatcatttaaatgatttatttccttgtgttcaggcgattcctccttctttgttaacttattcaccttttctattatggtgttcacggatgcctgtttgctctgtagtttcttaacaaaatccttaacttgtgaaaccatgttctgtgcaatgttcagctccagctcagagtgcctcctcttcatgttctgcagttgctgatcagcatcttgcaggtaaatccagagctcagacttcaggtgcttgatctcttcccagccctgagttaagttctgggcctggacaagcttttgttcaatcgtttgctctgtttgttgaatgtcttttgctgtggttttcaccgaagcatttgacaggtcacacatggagcaaaggagatctaggtaggtccttgcctgctcttgcaaagctctgaagtgtttgacctgcttaatggcttctgccctactaagaggtggttgaggacttggctctaaatccggctggactgcagaaagccaggcctggcactgctgcagggtgtcttgtcggctgacgtgcttctgaagttcgtgttccaaactctggtacatcctctgagctgtgctgcagatcgctgagtagctgtcctttgtgccctgcagatgagcatgcacgttttgtttaagtttcgcttgcaggtggtctgcacattggccaatcaaagtatcacctttcatttgaagattgttcaaacggtcttcaaaaccagcaatttcttccatcattgccttgtggtgggccaattgctgggtgattgtctccaggctgcttgtctccaggaggtcaggtgccaccagtctgccagacatctgcagcagccacttttcgacctcttggagctcactgttgtagtcttcatggtctttgactttcgcctccagactgaagacatgctcctttcctatgctgcacaggtcctggtaatcactttgaagttgatctattttgtcctttaaagtgacgtcctgcaccagttccaaaagagcttcacccttctctctcactgactttactgatggttcatgggacagcaccgtttgttgaagtgacttgtatttagataactgagcttttttctcatataattccattttgggttcttcaggaacatgtagaatttcctggtattctgctatccactgtgtcagtgctttgcatttatctgagaattcctttgctaaatgaagacctttttccagcgtcatgtgttctttccggacagtgctggtcagttccttcaactgctccatgtgatcatgaatctcctttcttaacctctctgcctcgccttcctccaagtatttaacagccctctctcctttctcccgggctgatttcagcaaactgtgacctttctccatgtctttgagcaaaacctccaacgtcttcaatttcttccccatcattactgtatctactttgtcaatcttggtagccacattcttgaagtttttatgagtagagccataccaatcagaataggaactgagggatgattctgattcctccaaactctgaatctcctcctccaggaattttatttgttccagcacttggagaagcagggcctggtatctggaagtcagctgggtggcctggcaacccattctgctgttcacgtggctctcgtccagtatctcctgagctctagctcccacttcctcaacttcatctctgtatgcagtcacttcttcgtgccacttcttcatctgatgtaattgtatctccttggttgccctgttagactgacgtctggtcctgggactaactttctcctctgctgttttgagccattcatctacttgctgaaacttttgctccattagcctcaatttgttcaccacgttattgaactgagttcgagtctcggacagcctgtgctggtaagcctgccagtcttgccggagagactctaaagcccggtcctctgcctgtgggatacctgatgggatcacatcctctctggtgtgcagcactgagttcaacagggcctgcccctctgcacagtgtacctgtagctcctgaagatcacgcaatgttgtctcatgagtgtgggcatcaccttcaagaactgaatactggtcgagcttttcttgttcttgccccaaccaaacttcaaatgcctttaggtctctctgatactcttggtgcaggcggacaagtttttcagacttggttacggcttccttggccctctcttggatggctctgtatcgttcctgtagatcctggagttctagctgggtgacatagtgttctgtcatgccagcccctttgacttcgatggtctccagcaagctgctgtaactcagcacttcttcatttaataacttggcttttccgagcatcgttgttttatcccgcagctccgcatgctgcctttctgattcattcaggttggcttccatactatccatccaaccggagaactgtcgaacgccatcctgataacttgtccacttggagagagctccttcgagttggcttttacaacgaatccctgcagacaaaagggatgcccacatatccttcacactctgcagctgctgctgaatagtgggaatgccttctggagaagtattctgaaggacagattctcccctggtcactatcattttcatctgaatctctttttcctgtttgactgataatagagcctcgagcttgagcgtcctgctgtccagcacacttttgtcggatgtcgggtggcagtatgaatccagcatgtgaatcgcatccgtcatccagtcttgtaattctttaatcccaagagagaactgattgtgttctgcaacgattctatccagtcttgacactttctcctttgttaaattgcttagcgctagatactgagaagacagctgcgacactctgtgcctaaagctcttgctggcagcttgtccttcccacagctgctgagctttctctttcagcctgttgagctgaggctcgtagcagtgtatttcctcaaggacagactggagcttctgctgctccctcctctttgctggcagatcatagaggcgattgctgctttcatggaccatcttctcagttttactcagccagtcctggataggctcagcacttacttcaaagtccttcatttggatctttagattctctagagcagattctttttggtggagatttgaatgaaaatttttccaatcttcttttgcagctgtaactttggcctggatccctttcgctttctctttggtcagcagggtactcagaagttcccctttagacagcatcatgtttagcttgtgctgtccattttcactttctgacaaaaactcctgtattttctgaagactagttgaaacttcacttatattttgaggtatatcaaaacacttggcggtagtgatttttgcattaaccaaccactgctggaaatccctgaaggcctttcgaaatctttgctgtaaaatctgttctttattctggcagcccttggatgcttgcaaacaaagacaattatactctttaatcaagccagaaacttttccactgtaggtactcaggtctctggaaaatcgacaaagttcattcagctgagacttgagatcctctgttctaggctctgctttttgcaaagcatccagtatctcttgtcctttgtgccagcattccactatctcctcatccgtgttcttgccttccaggagggttaactgctgagcccaggttttcagaagggcactgaactgttccagggcctgctccagttgagccacttggcctgagaattcctgctccgaaagggccatctggctgaccaggttctccaaacagctctgcgtttggaatacactgtcttcccactgcttccagtcggcacgcagggcctgcatctccgtgtgcatgagctcacacccactggcagttgtgttctgtttcacttcgggagccagcgactccactctgctgagacggcttgcaccaatctctctggaatctatcagctccttaatttttgataactttttctgggtggctgatgaatctccagacatatctgaccaccggtgaagttcttcctttgctgaatggagccaatctgtgaactcgtggaccgcatctaaatacattagatgatctttcacaatctcttccactttcctcattttttccttggcaacagtcattatatcattaaactgtgttttcagctcctcttgagctgtgtccttgaaagactcatcctctgtcttttcgtagagctccctggacttcgcaattagacggtgaagggctctcgtgtgatcttctgcctcagacaggatggactggaggtggtcaagcaggacgaacttctctttcagacctggctgtggttgtaagggatgttctattttttgatccactgattccatccactgctccaactggtttttcctctctacatagtcattccattggctaatcacagactctaaagtgctttgagcgtggacggaggagctcatgatgtcagcccacacttctttaagggtctctaactgagtctgaatcaccctctgaccttctttgttgctacttctcaaggcctgttcccccttgccaatggccatattcaacttaacttccccttcacctttcatcaggagaatatcctgtatttgtgacagccgtttctccagggtgtctttgctcccaagagtgctctctgcacaggccagtctgtcctgaatggccttcacccagaaccacatgctttgcagtgcttcctccagggcttcgtgctcctgaagggccacctggcagctccggagtttctctttggtcattctaagtaggttctggtggcttgtgaggagctgggaacacaggcggccctcctgcccagcaccgtggccttcttcactcagaagctgccctctctgggaaagcttatcaagagactctcttgcagccagcagttctcccaaaaacatttcaactttatgaacttcatttttcttctcaggaatgtgctgtttactctctcccaagttttccgtattgaacctttcttccatttcatggatccataagttcagttttctgtgctgatcttcaaagcttccaagttctgaagcacagtcttgaagagcctgcttatctttaaggcattgtttcagaaatgcttgaaactcttcattggcctttgtgatttgttcttgaatgctactgacaatttgtttagacaaatgtgcatacaaagtttgtccttcttgagtcactgcatcaagtttgctctgcccatcactgactgagtccaaaatgttctgaagatcatggagctttgcttctagaactttgctgtcaccggtgcgatctgatgattcttttgctgctgcctttgctcccaaaaaccattcttggaattcctgcatagactcactgaagtgtttttccagagattcctgcaggctggcctgggttttggagcacaactggctcacggcttcatgtttctttatcagaccagtcattgcacggcccaggctctccaactcagctgagtggtacttgcggcacaagctattgagattttcttgggtagagctgatgttgctttgttgactttgaagttctttttgtatatccttgacttttttcaatgcttcacaagtctcattttgggcacagttcatcaacgattcttccacttttgtgaaccatgttgttatgtcattaataaacttctccacttgtgtactttgagccgtgaaatccttcagggttccttttgctacttcagttatttctttggcatgctccagtttctgcattaagtctgcttctataaactgaaggtctggcggtgtttctagatttttagttaattctttcagatcattaactttggaatgcagttcttccaatctcaatgctttgtttttaacttcagactcaaattctttaagcagttcttcagctctgaggtggttatccaggttgctgatgttttctgccatctgtggaacgcagttgtttgaccatccctcaatctcatctctagttgacagtacatcatcccaaatggacaggcttactctcagcctatccatgttttcttcaagtttctctgatacatccagccatttgtccacggtgctctccatgtctgttttcaccaagctgaaatcactactgtgaattttcttcagctcagataacaagtgttttcctttgctggtaaagttatccaagtctttctgtttgtaattcattttgttcttggcagtttcatgcttggaaaaagcccatttaagatcctcctgatcttttatggtagttctggttacaatcacactgctggcattttctaagactttagatacagctgatttcaggttctgatattctctcattaagtcaataagtccacagcactgaccctgattttcatgaattagtcttttggtatcatcccaggtgacctctaagcggtttatctccctgtcaacttcaggtgcaaaagctacatctttctgggcaatttgcttggctttgtctttcaaccaacatagttcatgctcgtgagaattcaattcatcttctagctgattaaacactcttaacctctgctgaagagcttggcgggtaggttctttcaatcgctctttgtcagtcctttcttcaatgtcctcaatgcttttcagaagctcctctttctggtcttggaatgcttttttcaacactgccagagcatctgcctcactctgcttggttcccagaaggttctggatcctctctacctctccacagagctgatcagccgtggctctgcaggaagtcctttgctcagagctcccgattttcagatggtattgggctttggaaagaatgccatccagactgacggcagcagattctaatgctttagcattttgaagagcatcattgaggtccttttctatcaaatcagactcgttcttattcatactgttggttgcttccactgtttgcctcagctggcggagaatgccggacagagaggcatggctctggaggaattctgccaaatgggacagggcaagctgccgcctctccacaacctggctggcctcctcaaacagctggaagcagtcctcagcctttccctgcaggaggtggaggtcctcagcacggcccagagaacccaactttgctaagtgaccctgcagactctgcaattcgccctttttgctctctacttctgctgcgtggtccttatgccgagtaagggctacttgatggtccattatgctaatctcagaggtagtttgtaattcactgagaaacagtttaatccagacagaaaaggaaagcagcagctcatcaaattgctggtgttcagcaaccacagactgaagaaaattaatccttttgttaatgatctgtggtaaatctctccatctctcatccaactgctccaaatgtagtttcatcattttcacatcatctttggaggctactgagaacaatgattccttcaattgcaaaagtttgctatagaatgaggcctgggatacaacttcattttgcagtgcctgtattaactgaagttcaccttccactttgactctgtctgcagaaatgtccatttctggggaactggctttagcttcaccccgctctaaccaggtcaaaaaggatgatagttctttctctagcctctgccagtgggccagcagattctccagcgccgtctgtctctccttcgccctccttaggatgtcctcgtattgctgctgtagagccgcagcctcctgaacacaggaatctctgttcacaaccttcctggcactggctgagaaggcagtgatcgcgctgctcagtgactccagggcctggcagagatccatatgttcttgaagaactttgtatgtttctgtagctgaagaacatattttaattggaacagcaagtttatcttcaaattcagacacagattgctggatctttctaaggttctcttcaaacttttgctgctgagataaatgtcccaggattgttccttccagacactgtgcatgctctcgaagctcttccccgtatcttcttatttgtgtcaacttggctttaattcgagcagattctccagtggtaacaaactgagcaaaagactgggcttcttcttctaatcctacaatgctgctgagcttactttctatttcctgaattgtgaccttaatttggctgatttgcatgtccatggcagatgacgaagtttccaaggcattgagttctttttctttctcagttatccagacggacagagtctcaaaattactgccaaaatgatcccacttggttttcaccatttccatggttttaatatcttcttcaagcgtgtcttctaattttttgacttgttctttgattgacttggcctgctgttgaagcagctgcttattttggggcccaagcggtatctctgaagcttcctttacaaggttctcagcctggactgcaatactttctgtccgtttagaaaactcctttgtttgttccagttctgaagataaactttccaaactgctaaaactcaagaagcgttcatgactggaacctgtttgaaaaaggtatcttactactgtttctttgtttgtttcaaatcgctcccattttcttaatgtgacctggatgcggcgttcctgcctctcccggctgcgctccaggccatccagtgtgctctccagcttccgcagctcctcgtggcctcggtcaggcagccccccttctccctgctgcgcctgcgcgatctgctgctgcacatctctcttctttgctgagatccgctttgtcttttgctggtgatgaagaagtaactgctgtgcttcaaacagattttcagtatccaagatcttctcagcttgttcctggacttctttagagccagaaattaattcttcgagagaatttttgactatttctttgtactggacacagtccccaaaattgcttagcatcttttcaacctctgacagcagcgtcacaagagccttgaaagagctggataattttgccagctcatctccctgcttttgggcttcattctcagaagaaacttctgtcaaaactttcagcctggatttcagccagctgagggtctcaccccttttggtaacaccatttctgatctcttcaacggcacgtttaacctctccgtggttggcagtatcgatggcctcacccttgatcccctttaattgtgtctcatttgtagatatccaagatgagaactcagagaatctgctagtgtagtccttccacttgtctgggtcttccatgagcttcctgtaggtgctgtcaatggcagctctgagctctttgagagtcacgtgacaggttccaggtgtgtcccttactgggtcccgcactgggagtttcacacagagttcctcgatgagctgtaaccttttctcacagagatgatgaggacctttgtcactgaagaaaaccctgtgctctttaattatcttttcactgccttcctggggcatcagcttggtctctcgatccagctcagttctgcattcttctacagaggctaagaacctattcttctccacatcaatcttcagatgaagcaaatgataaggggcttctccttgaagatccttccattgtttgtggagctttcgaacagcttcctgcagcccctgctgctcctgctctggaaggatgtcggtgagttcatcacaagctttcaggaaagcattgagcaccctctgatccagctgactgaaaaactcagtgtgtctccgcaggagctcctctggatcccccttttcctccaggccctcctgagcaatccgcagtaccttctccaactctgctcgagactcctcaaacttcttcatcaagcgactgttggtttccacatgcttcttccaatctccagttttctttaccatactctgaaaagcaacatgaatatctgcaatctgtctttgtagcctcgtctgatcaaaatgctttaacacgttgctcaaggtcacaaacttttgaacactttgactgcctttctcaataagtgtcaaggttttcttacagttttcttgacaagctaacagttcctgatgtttttgtttaaaaagggcactcgattgtgcctcacgctcaagaactgtgataatttcattgattttcccaagtgagtcataaaaggacgtcatctgcttttctaattcctccaacggaatcaacagctgctgagactcataaaggagtggggagtaacattctttgaccttggttagctgctctttgagctttgacatggtcgcaaacatttcttttccttcttcttgggggctttctttggtaatgaggtgtgctgtctttgtaattatcttgtattgggcatccatcacaggcaccctctgctcaatatcctccaagtcttgaattaatagcttgacattcataaaagagacttctaagggttcagaaagtttcttatgggcttccgttgcaaaagcagacagggtaacaacacagtctgtgtattccttcttcattctgtccatctcatcagcttgagcatattgcttgacttccataaacaactccctccaccgcccatttagcaacagtaattgctgcttcaggtcacgggaaaccatctcatcacaggtttcaattagaaaattgccagcatcgttcatggcagtatgctgctgaatccaatgaggtaaatttcgaaaaaaatcctttttggcattttctgattgattgagcattttttcagcatcctctagccaggcttgcagactagccactgtattgccatagcgatcccagttagagatcacttcttccagcatgctcctcacactcctcacttctactgagagattcctccactgagcggtggtttcattcatgaatttcatcacattctcagcttcttccactgaaccatctgctttgacatacatctcagctgtctgtttcaagatctggtatgtcacctcatattgttcaaagaacttgctattttctataaaagacacgtagttttgtagaagctgctccactgactctctcctcccgtacttaatgatccaagacttcagctttgactctgcaagaaccagcagtgagagcagacggtactttaattctaaaaattccattttcattaggtgtagctctgatgtggaggaaacaaaatgaaacctctcggccatgtcctctaattgatcaggtggcactggaatcccgttaacagacctggtccggtagatttcatggaatgctcttttgtgggcatccgtgttttgaagcagatccttatgttgctcaagtttccgttgtatcgtgtttgctgtttcctcgtggacctgttgaacggttatttcctctctcagggccacctccgctctgtacagccaggcacctatggtgcccagaggtgcaggaagagatttatcaagctgtatatgccagtcaaagagcctggaggtcactctatcccaagattgttttaccaatgcttggtcaagtgacaatttaccgtctctgtgtaatggttgtattaaatgttcaatctgtttcctcttcatttcatattgaactctgaagtgcttaaatgactgatatttatcctgtaaatttgattccaccatctgtgctcttgtcaaatctctctcaaattgttctatccaaactttcatttccttaaaaattactctgtcttctctatcatcctcttgcccatcagtgcttgcattgtggatgtcaggataatgtttcagaaactgggctacataggtcataatagatttctcatctggtttatccacatcaacgtcttcaggatctagcagtcttgggatccccagttctgtttcggcgatagtgaaagcatcctccaaattttctcggttggatctgcctttcactgtctccaagtccaccaattccggtcgaatggcatgaataactgaatgaaaggcaaccccgcttctccaactcttcccaaaatcttttacttctattccagtctgcttgccagctgtgtactgaacccactttaataaagccttcttagcatttccttggatcttggtggtcaccttccgtttacttggtgggctgggagtctcagagctaactatgctgtccacggaggatgcgctgctggacaaagactggagctggggcaggttgctggtcaactcttcaatctggaaatatagaataatggtccacatcaatccaagaactattgagggtcggccatcagctatatcggtggagttaatgttgactaatttaatcggtgatcctctgtgcatggactttcttccttcgaggaacttgagtgccgtgccaatgttagccacagcatggattcgcttcatccggcgtccttgttcacaaggcagtttctgcccagacaggacctccagaagggcaagcagtttaacaccatctttcatgtcttcaaaaagatcgtccaccaccattggaggtttccgcttggccagatgagagttgatccattttgtgaaagttcgtttttgtactatctcttgctcatcttgcagcctctgcatcacattggcgatatcccgaggacaccgggaggcccctctggaggttgccatggtccctccggaagcacgaagccaacaccaagagactcttcactggaggcagcacagggctacaccactctagaaaacatgcttggacttttctagatctattctgtcataaatgaattccaggcctttgcagcactcaacaaggaggcagctctcccaaagactgaactgcttctttttcttcttccgttttaagactgtcctcttacatgaactcaagaaccttctctctcggcctcgttcagtttcccagcagcaaggcgaagcgagcgaacgcttcctcccggctctctgcgcccaggctcggcgggaccccggggatgcgcggctgtccgcccgccctgtcgccgggatcgggcgcggtctgcaggactgcgggagcccagccgccctggtgacagaggacaacaatctcagcccgctgcggccggcggccgcggcccggcgcccgcgctcaccctggctggctcgcccacact

SEQ ID NO: 9568 - RNA, 13869 nt, Homo sapiens
  source 1..13869: mol_type = other RNA
agttcttcagtggcaagctttatcaaaatcttccttaaaatgcttcctagaaaccaaattcttctctagttcttgtaaccggtgactgcacttttgtaaaacactgtcatagacactctgcaattcctgaagcttccccagcacttcactcttttcctgctctgtgacttccttcattagttcgcgaccctgggcccaaagtccagtgacttcattttggtaagtcttgaggctggcttgtgcactcttacatgttttgacttgtttgctcacatcatctggtaacagacagatgtgttcacggaacattatctttcgctcatgttgctgaatttggctggtggcctggaacactgccatgagaaactgggttttctcggacaaggctttgtttaagtactttcttcgctggcccactaagtcactgagacaattcacgtggctttgtgcatcagagagagccttctggatgacctgtcgctcattgagaccaagatctgccatgaccctgtctgcgtcctttataagcgatttcaggagcatctgcttggcctccagttcactgcagatggccaggtgatccatgagaaggttctgagccatatctggaggagggctctgcttaagggcctcggcgatgttgggttgttgctcttctgcccactccattagctcctgaaatctggactgcaccacatttaactcctccaagttggtgactgacacttggattttccttttaatgaggtcctcaagctgaaaccaacgttgctctaaatgactcgtctgttctttgactaactccttgtcatctaaattcagatgctctatcattttctgcttttgatctttcagatcttcaatagcatactttctctcctgcaatgccaatgctaactttttcaaagcttccaggtggacagctgtactctctgcatcagatctggccaagttatcccattctgtagtaaatttttctaggaacacttcaacaacattcatacagtcatggtaatctcttgttctctgaagatcctcttccctttgcaagcacaggttgttagactgacggcacaaatcgagccactgatcatttaaatgatttatttccttgtgttcaggcgattcctccttctttgttaacttattcaccttttctattatggtgttcacggatgcctgtttgctctgtagtttcttaacaaaatccttaacttgtgaaaccatgttctgtgcaatgttcagctccagctcagagtgcctcctcttcatgttctgcagttgctgatcagcatcttgcaggtaaatccagagctcagacttcaggtgcttgatctcttcccagccctgagttaagttctgggcctggacaagcttttgttcaatcgtttgctctgtttgttgaatgtcttttgctgtggttttcaccgaagcatttgacaggtcacacatggagcaaaggagatctaggtaggtccttgcctgctcttgcaaagctctgaagtgtttgacctgcttaatggcttctgccctactaagaggtggttgaggacttggctctaaatccggctggactgcagaaagccaggcctggcactgctgcagggtgtcttgtcggctgacgtgcttctgaagttcgtgttccaaactctggtacatcctctgagctgtgctgcagatcgctgagtagctgtcctttgtgccctgcagatgagcatgcacgttttgtttaagtttcgcttgcaggtggtctgcacattggccaatcaaagtatcacctttcatttgaagattgttcaaacggtcttcaaaaccagcaatttcttccatcattgccttgtggtgggccaattgctgggtgattgtctccaggctgcttgtctccaggaggtcaggtgccaccagtctgccagacatctgcagcagccacttttcgacctcttggagctcactgttgtagtcttcatggtctttgactttcgcctccagactgaagacatgctcctttcctatgctgcacaggtcctggtaatcactttgaagttgatctattttgtcctttaaagtgacgtcctgcaccagttccaaaagagcttcacccttctctctcactgactttactgatggttcatgggacagcaccgtttgttgaagtgacttgtatttagataactgagcttttttctcatataattccattttgggttcttcaggaacatgtagaatttcctggtattctgctatccactgtgtcagtgctttgcatttatctgagaattcctttgctaaatgaagacctttttccagcgtcatgtgttctttccggacagtgctggtcagttccttcaactgctccatgtgatcatgaatctcctttcttaacctctctgcctcgccttcctccaagtatttaacagccctctctcctttctcccgggctgatttcagcaaactgtgacctttctccatgtctttgagcaaaacctccaacgtcttcaatttcttccccatcattactgtatctactttgtcaatcttggtagccacattcttgaagtttttatgagtagagccataccaatcagaataggaactgagggatgattctgattcctccaaactctgaatctcctcctccaggaattttatttgttccagcacttggagaagcagggcctggtatctggaagtcagctgggtggcctggcaacccattctgctgttcacgtggctctcgtccagtatctcctgagctctagctcccacttcctcaacttcatctctgtatgcagtcacttcttcgtgccacttcttcatctgatgtaattgtatctccttggttgccctgttagactgacgtctggtcctgggactaactttctcctctgctgttttgagccattcatctacttgctgaaacttttgctccattagcctcaatttgttcaccacgttattgaactgagttcgagtctcggacagcctgtgctggtaagcctgccagtcttgccggagagactctaaagcccggtcctctgcctgtgggatacctgatgggatcacatcctctctggtgtgcagcactgagttcaacagggcctgcccctctgcacagtgtacctgtagctcctgaagatcacgcaatgttgtctcatgagtgtgggcatcaccttcaagaactgaatactggtcgagcttttcttgttcttgccccaaccaaacttcaaatgcctttaggtctctctgatactcttggtgcaggcggacaagtttttcagacttggttacggcttccttggccctctcttggatggctctgtatcgttcctgtagatcctggagttctagctgggtgacatagtgttctgtcatgccagcccctttgacttcgatggtctccagcaagctgctgtaactcagcacttcttcatttaataacttggcttttccgagcatcgttgttttatcccgcagctccgcatgctgcctttctgattcattcaggttggcttccatactatccatccaaccggagaactgtcgaacgccatcctgataacttgtccacttggagagagctccttcgagttggcttttacaacgaatccctgcagacaaaagggatgcccacatatccttcacactctgcagctgctgctgaatagtgggaatgccttctggagaagtattctgaaggacagattctcccctggtcactatcattttcatctgaatctctttttcctgtttgactgataatagagcctcgagcttgagcgtcctgctgtccagcacacttttgtcggatgtcgggtggcagtatgaatccagcatgtgaatcgcatccgtcatccagtcttgtaattctttaatcccaagagagaactgattgtgttctgcaacgattctatccagtcttgacactttctcctttgttaaattgcttagcgctagatactgagaagacagctgcgacactctgtgcctaaagctcttgctggcagcttgtccttcccacagctgctgagctttctctttcagcctgttgagctgaggctcgtagcagtgtatttcctcaaggacagactggagcttctgctgctccctcctctttgctggcagatcatagaggcgattgctgctttcatggaccatcttctcagttttactcagccagtcctggataggctcagcacttacttcaaagtccttcatttggatctttagattctctagagcagattctttttggtggagatttgaatgaaaatttttccaatcttcttttgcagctgtaactttggcctggatccctttcgctttctctttggtcagcagggtactcagaagttcccctttagacagcatcatgtttagcttgtgctgtccattttcactttctgacaaaaactcctgtattttctgaagactagttgaaacttcacttatattttgaggtatatcaaaacacttggcggtagtgatttttgcattaaccaaccactgctggaaatccctgaaggcctttcgaaatctttgctgtaaaatctgttctttattctggcagcccttggatgcttgcaaacaaagacaattatactctttaatcaagccagaaacttttccactgtaggtactcaggtctctggaaaatcgacaaagttcattcagctgagacttgagatcctctgttctaggctctgctttttgcaaagcatccagtatctcttgtcctttgtgccagcattccactatctcctcatccgtgttcttgccttccaggagggttaactgctgagcccaggttttcagaagggcactgaactgttccagggcctgctccagttgagccacttggcctgagaattcctgctccgaaagggccatctggctgaccaggttctccaaacagctctgcgtttggaatacactgtcttcccactgcttccagtcggcacgcagggcctgcatctccgtgtgcatgagctcacacccactggcagttgtgttctgtttcacttcgggagccagcgactccactctgctgagacggcttgcaccaatctctctggaatctatcagctccttaatttttgataactttttctgggtggctgatgaatctccagacatatctgaccaccggtgaagttcttcctttgctgaatggagccaatctgtgaactcgtggaccgcatctaaatacattagatgatctttcacaatctcttccactttcctcattttttccttggcaacagtcattatatcattaaactgtgttttcagctcctcttgagctgtgtccttgaaagactcatcctctgtcttttcgtagagctccctggacttcgcaattagacggtgaagggctctcgtgtgatcttctgcctcagacaggatggactggaggtggtcaagcaggacgaacttctctttcagacctggctgtggttgtaagggatgttctattttttgatccactgattccatccactgctccaactggtttttcctctctacatagtcattccattggctaatcacagactctaaagtgctttgagcgtggacggaggagctcatgatgtcagcccacacttctttaagggtctctaactgagtctgaatcaccctctgaccttctttgttgctacttctcaaggcctgttcccccttgccaatggccatattcaacttaacttccccttcacctttcatcaggagaatatcctgtatttgtgacagccgtttctccagggtgtctttgctcccaagagtgctctctgcacaggccagtctgtcctgaatggccttcacccagaaccacatgctttgcagtgcttcctccagggcttcgtgctcctgaagggccacctggcagctccggagtttctctttggtcattctaagtaggttctggtggcttgtgaggagctgggaacacaggcggccctcctgcccagcaccgtggccttcttcactcagaagctgccctctctgggaaagcttatcaagagactctcttgcagccagcagttctcccaaaaacatttcaactttatgaacttcatttttcttctcaggaatgtgctgtttactctctcccaagttttccgtattgaacctttcttccatttcatggatccataagttcagttttctgtgctgatcttcaaagcttccaagttctgaagcacagtcttgaagagcctgcttatctttaaggcattgtttcagaaatgcttgaaactcttcattggcctttgtgatttgttcttgaatgctactgacaatttgtttagacaaatgtgcatacaaagtttgtccttcttgagtcactgcatcaagtttgctctgcccatcactgactgagtccaaaatgttctgaagatcatggagctttgcttctagaactttgctgtcaccggtgcgatctgatgattcttttgctgctgcctttgctcccaaaaaccattcttggaattcctgcatagactcactgaagtgtttttccagagattcctgcaggctggcctgggttttggagcacaactggctcacggcttcatgtttctttatcagaccagtcattgcacggcccaggctctccaactcagctgagtggtacttgcggcacaagctattgagattttcttgggtagagctgatgttgctttgttgactttgaagttctttttgtatatccttgacttttttcaatgcttcacaagtctcattttgggcacagttcatcaacgattcttccacttttgtgaaccatgttgttatgtcattaataaacttctccacttgtgtactttgagccgtgaaatccttcagggttccttttgctacttcagttatttctttggcatgctccagtttctgcattaagtctgcttctataaactgaaggtctggcggtgtttctagatttttagttaattctttcagatcattaactttggaatgcagttcttccaatctcaatgctttgtttttaacttcagactcaaattctttaagcagttcttcagctctgaggtggttatccaggttgctgatgttttctgccatctgtggaacgcagttgtttgaccatccctcaatctcatctctagttgacagtacatcatcccaaatggacaggcttactctcagcctatccatgttttcttcaagtttctctgatacatccagccatttgtccacggtgctctccatgtctgttttcaccaagctgaaatcactactgtgaattttcttcagctcagataacaagtgttttcctttgctggtaaagttatccaagtctttctgtttgtaattcattttgttcttggcagtttcatgcttggaaaaagcccatttaagatcctcctgatcttttatggtagttctggttacaatcacactgctggcattttctaagactttagatacagctgatttcaggttctgatattctctcattaagtcaataagtccacagcactgaccctgattttcatgaattagtcttttggtatcatcccaggtgacctctaagcggtttatctccctgtcaacttcaggtgcaaaagctacatctttctgggcaatttgcttggctttgtctttcaaccaacatagttcatgctcgtgagaattcaattcatcttctagctgattaaacactcttaacctctgctgaagagcttggcgggtaggttctttcaatcgctctttgtcagtcctttcttcaatgtcctcaatgcttttcagaagctcctctttctggtcttggaatgcttttttcaacactgccagagcatctgcctcactctgcttggttcccagaaggttctggatcctctctacctctccacagagctgatcagccgtggctctgcaggaagtcctttgctcagagctcccgattttcagatggtattgggctttggaaagaatgccatccagactgacggcagcagattctaatgctttagcattttgaagagcatcattgaggtccttttctatcaaatcagactcgttcttattcatactgttggttgcttccactgtttgcctcagctggcggagaatgccggacagagaggcatggctctggaggaattctgccaaatgggacagggcaagctgccgcctctccacaacctggctggcctcctcaaacagctggaagcagtcctcagcctttccctgcaggaggtggaggtcctcagcacggcccagagaacccaactttgctaagtgaccctgcagactctgcaattcgccctttttgctctctacttctgctgcgtggtccttatgccgagtaagggctacttgatggtccattatgctaatctcagaggtagtttgtaattcactgagaaacagtttaatccagacagaaaaggaaagcagcagctcatcaaattgctggtgttcagcaaccacagactgaagaaaattaatccttttgttaatgatctgtggtaaatctctccatctctcatccaactgctccaaatgtagtttcatcattttcacatcatctttggaggctactgagaacaatgattccttcaattgcaaaagtttgctatagaatgaggcctgggatacaacttcattttgcagtgcctgtattaactgaagttcaccttccactttgactctgtctgcagaaatgtccatttctggggaactggctttagcttcaccccgctctaaccaggtcaaaaaggatgatagttctttctctagcctctgccagtgggccagcagattctccagcgccgtctgtctctccttcgccctccttaggatgtcctcgtattgctgctgtagagccgcagcctcctgaacacaggaatctctgttcacaaccttcctggcactggctgagaaggcagtgatcgcgctgctcagtgactccagggcctggcagagatccatatgttcttgaagaactttgtatgtttctgtagctgaagaacatattttaattggaacagcaagtttatcttcaaattcagacacagattgctggatctttctaaggttctcttcaaacttttgctgctgagataaatgtcccaggattgttccttccagacactgtgcatgctctcgaagctcttccccgtatcttcttatttgtgtcaacttggctttaattcgagcagattctccagtggtaacaaactgagcaaaagactgggcttcttcttctaatcctacaatgctgctgagcttactttctatttcctgaattgtgaccttaatttggctgatttgcatgtccatggcagatgacgaagtttccaaggcattgagttctttttctttctcagttatccagacggacagagtctcaaaattactgccaaaatgatcccacttggttttcaccatttccatggttttaatatcttcttcaagcgtgtcttctaattttttgacttgttctttgattgacttggcctgctgttgaagcagctgcttattttggggcccaagcggtatctctgaagcttcctttacaaggttctcagcctggactgcaatactttctgtccgtttagaaaactcctttgtttgttccagttctgaagataaactttccaaactgctaaaactcaagaagcgttcatgactggaacctgtttgaaaaaggtatcttactactgtttctttgtttgtttcaaatcgctcccattttcttaatgtgacctggatgcggcgttcctgcctctcccggctgcgctccaggccatccagtgtgctctccagcttccgcagctcctcgtggcctcggtcaggcagccccccttctccctgctgcgcctgcgcgatctgctgctgcacatctctcttctttgctgagatccgctttgtcttttgctggtgatgaagaagtaactgctgtgcttcaaacagattttcagtatccaagatcttctcagcttgttcctggacttctttagagccagaaattaattcttcgagagaatttttgactatttctttgtactggacacagtccccaaaattgcttagcatcttttcaacctctgacagcagcgtcacaagagccttgaaagagctggataattttgccagctcatctccctgcttttgggcttcattctcagaagaaacttctgtcaaaactttcagcctggatttcagccagctgagggtctcaccccttttggtaacaccatttctgatctcttcaacggcacgtttaacctctccgtggttggcagtatcgatggcctcacccttgatcccctttaattgtgtctcatttgtagatatccaagatgagaactcagagaatctgctagtgtagtccttccacttgtctgggtcttccatgagcttcctgtaggtgctgtcaatggcagctctgagctctttgagagtcacgtgacaggttccaggtgtgtcccttactgggtcccgcactgggagtttcacacagagttcctcgatgagctgtaaccttttctcacagagatgatgaggacctttgtcactgaagaaaaccctgtgctctttaattatcttttcactgccttcctggggcatcagcttggtctctcgatccagctcagttctgcattcttctacagaggctaagaacctattcttctccacatcaatcttcagatgaagcaaatgataaggggcttctccttgaagatccttccattgtttgtggagctttcgaacagcttcctgcagcccctgctgctcctgctctggaaggatgtcggtgagttcatcacaagctttcaggaaagcattgagcaccctctgatccagctgactgaaaaactcagtgtgtctccgcaggagctcctctggatcccccttttcctccaggccctcctgagcaatccgcagtaccttctccaactctgctcgagactcctcaaacttcttcatcaagcgactgttggtttccacatgcttcttccaatctccagttttctttaccatactctgaaaagcaacatgaatatctgcaatctgtctttgtagcctcgtctgatcaaaatgctttaacacgttgctcaaggtcacaaacttttgaacactttgactgcctttctcaataagtgtcaaggttttcttacagttttcttgacaagctaacagttcctgatgtttttgtttaaaaagggcactcgattgtgcctcacgctcaagaactgtgataatttcattgattttcccaagtgagtcataaaaggacgtcatctgcttttctaattcctccaacggaatcaacagctgctgagactcataaaggagtggggagtaacattctttgaccttggttagctgctctttgagctttgacatggtcgcaaacatttcttttccttcttcttgggggctttctttggtaatgaggtgtgctgtctttgtaattatcttgtattgggcatccatcacaggcaccctctgctcaatatcctccaagtcttgaattaatagcttgacattcataaaagagacttctaagggttcagaaagtttcttatgggcttccgttgcaaaagcagacagggtaacaacacagtctgtgtattccttcttcattctgtccatctcatcagcttgagcatattgcttgacttccataaacaactccctccaccgcccatttagcaacagtaattgctgcttcaggtcacgggaaaccatctcatcacaggtttcaattagaaaattgccagcatcgttcatggcagtatgctgctgaatccaatgaggtaaatttcgaaaaaaatcctttttggcattttctgattgattgagcattttttcagcatcctctagccaggcttgcagactagccactgtattgccatagcgatcccagttagagatcacttcttccagcatgctcctcacactcctcacttctactgagagattcctccactgagcggtggtttcattcatgaatttcatcacattctcagcttcttccactgaaccatctgctttgacatacatctcagctgtctgtttcaagatctggtatgtcacctcatattgttcaaagaacttgctattttctataaaagacacgtagttttgtagaagctgctccactgactctctcctcccgtacttaatgatccaagacttcagctttgactctgcaagaaccagcagtgagagcagacggtactttaattctaaaaattccattttcattaggtgtagctctgatgtggaggaaacaaaatgaaacctctcggccatgtcctctaattgatcaggtggcactggaatcccgttaacagacctggtccggtagatttcatggaatgctcttttgtgggcatccgtgttttgaagcagatccttatgttgctcaagtttccgttgtatcgtgtttgctgtttcctcgtggacctgttgaacggttatttcctctctcagggccacctccgctctgtacagccaggcacctatggtgcccagaggtgcaggaagagatttatcaagctgtatatgccagtcaaagagcctggaggtcactctatcccaagattgttttaccaatgcttggtcaagtgacaatttaccgtctctgtgtaatggttgtattaaatgttcaatctgtttcctcttcatttcatattgaactctgaagtgcttaaatgactgatatttatcctgtaaatttgattccaccatctgtgctcttgtcaaatctctctcaaattgttctatccaaactttcatttccttaaaaattactctgtcttctctatcatcctcttgcccatcagtgcttgcattgtggatgtcaggataatgtttcagaaactgggctacataggtcataatagatttctcatctggtttatccacatcaacgtcttcaggatctagcagtcttgggatccccagttctgtttcggcgatagtgaaagcatcctccaaattttctcggttggatctgcctttcactgtctccaagtccaccaattccggtcgaatggcatgaataactgaatgaaaggcaaccccgcttctccaactcttcccaaaatcttttacttctattccagtctgcttgccagctgtgtactgaacccactttaataaagccttcttagcatttccttggatcttggtggtcaccttccgtttacttggtgggctgggagtctcagagctaactatgctgtccacggaggatgcgctgctggacaaagactggagctggggcaggttgctggtcaactcttcaatctggaaatatagaataatggtccacatcaatccaagaactattgagggtcggccatcagctatatcggtggagttaatgttgactaatttaatcggtgatcctctgtgcatggactttcttccttcgaggaacttgagtgccgtgccaatgttagccacagcatggattcgcttcatccggcgtccttgttcacaaggcagtttctgcccagacaggacctccagaagggcaagcagtttaacaccatctttcatgtcttcaaaaagatcgtccaccaccattggaggtttccgcttggccagatgagagttgatccattttgtgaaagttcgtttttgtactatctcttgctcatcttttatcatacccggagtcttgtagattgtttttatcatatctcacctattttactgattttggtaaattatcctaattcagtcgtatctaaaccaaacacagctttcaccaagggaacttccaactctcctagcagcattctcctgatattatcactatagcaacatctctataaaagcatactattcttccctcattcttcatccttaccccctgcttactagcca

SEQ ID NO: 9569 - RNA, 14165 nt, Homo sapiens
  source 1..14165: mol_type = other RNA
agttcttcagtggcaagctttatcaaaatcttccttaaaatgcttcctagaaaccaaattcttctctagttcttgtaaccggtgactgcacttttgtaaaacactgtcatagacactctgcaattcctgaagcttccccagcacttcactcttttcctgctctgtgacttccttcattagttcgcgaccctgggcccaaagtccagtgacttcattttggtaagtcttgaggctggcttgtgcactcttacatgttttgacttgtttgctcacatcatctggtaacagacagatgtgttcacggaacattatctttcgctcatgttgctgaatttggctggtggcctggaacactgccatgagaaactgggttttctcggacaaggctttgtttaagtactttcttcgctggcccactaagtcactgagacaattcacgtggctttgtgcatcagagagagccttctggatgacctgtcgctcattgagaccaagatctgccatgaccctgtctgcgtcctttataagcgatttcaggagcatctgcttggcctccagttcactgcagatggccaggtgatccatgagaaggttctgagccatatctggaggagggctctgcttaagggcctcggcgatgttgggttgttgctcttctgcccactccattagctcctgaaatctggactgcaccacatttaactcctccaagttggtgactgacacttggattttccttttaatgaggtcctcaagctgaaaccaacgttgctctaaatgactcgtctgttctttgactaactccttgtcatctaaattcagatgctctatcattttctgcttttgatctttcagatcttcaatagcatactttctctcctgcaatgccaatgctaactttttcaaagcttccaggtggacagctgtactctctgcatcagatctggccaagttatcccattctgtagtaaatttttctaggaacacttcaacaacattcatacagtcatggtaatctcttgttctctgaagatcctcttccctttgcaagcacaggttgttagactgacggcacaaatcgagccactgatcatttaaatgatttatttccttgtgttcaggcgattcctccttctttgttaacttattcaccttttctattatggtgttcacggatgcctgtttgctctgtagtttcttaacaaaatccttaacttgtgaaaccatgttctgtgcaatgttcagctccagctcagagtgcctcctcttcatgttctgcagttgctgatcagcatcttgcaggtaaatccagagctcagacttcaggtgcttgatctcttcccagccctgagttaagttctgggcctggacaagcttttgttcaatcgtttgctctgtttgttgaatgtcttttgctgtggttttcaccgaagcatttgacaggtcacacatggagcaaaggagatctaggtaggtccttgcctgctcttgcaaagctctgaagtgtttgacctgcttaatggcttctgccctactaagaggtggttgaggacttggctctaaatccggctggactgcagaaagccaggcctggcactgctgcagggtgtcttgtcggctgacgtgcttctgaagttcgtgttccaaactctggtacatcctctgagctgtgctgcagatcgctgagtagctgtcctttgtgccctgcagatgagcatgcacgttttgtttaagtttcgcttgcaggtggtctgcacattggccaatcaaagtatcacctttcatttgaagattgttcaaacggtcttcaaaaccagcaatttcttccatcattgccttgtggtgggccaattgctgggtgattgtctccaggctgcttgtctccaggaggtcaggtgccaccagtctgccagacatctgcagcagccacttttcgacctcttggagctcactgttgtagtcttcatggtctttgactttcgcctccagactgaagacatgctcctttcctatgctgcacaggtcctggtaatcactttgaagttgatctattttgtcctttaaagtgacgtcctgcaccagttccaaaagagcttcacccttctctctcactgactttactgatggttcatgggacagcaccgtttgttgaagtgacttgtatttagataactgagcttttttctcatataattccattttgggttcttcaggaacatgtagaatttcctggtattctgctatccactgtgtcagtgctttgcatttatctgagaattcctttgctaaatgaagacctttttccagcgtcatgtgttctttccggacagtgctggtcagttccttcaactgctccatgtgatcatgaatctcctttcttaacctctctgcctcgccttcctccaagtatttaacagccctctctcctttctcccgggctgatttcagcaaactgtgacctttctccatgtctttgagcaaaacctccaacgtcttcaatttcttccccatcattactgtatctactttgtcaatcttggtagccacattcttgaagtttttatgagtagagccataccaatcagaataggaactgagggatgattctgattcctccaaactctgaatctcctcctccaggaattttatttgttccagcacttggagaagcagggcctggtatctggaagtcagctgggtggcctggcaacccattctgctgttcacgtggctctcgtccagtatctcctgagctctagctcccacttcctcaacttcatctctgtatgcagtcacttcttcgtgccacttcttcatctgatgtaattgtatctccttggttgccctgttagactgacgtctggtcctgggactaactttctcctctgctgttttgagccattcatctacttgctgaaacttttgctccattagcctcaatttgttcaccacgttattgaactgagttcgagtctcggacagcctgtgctggtaagcctgccagtcttgccggagagactctaaagcccggtcctctgcctgtgggatacctgatgggatcacatcctctctggtgtgcagcactgagttcaacagggcctgcccctctgcacagtgtacctgtagctcctgaagatcacgcaatgttgtctcatgagtgtgggcatcaccttcaagaactgaatactggtcgagcttttcttgttcttgccccaaccaaacttcaaatgcctttaggtctctctgatactcttggtgcaggcggacaagtttttcagacttggttacggcttccttggccctctcttggatggctctgtatcgttcctgtagatcctggagttctagctgggtgacatagtgttctgtcatgccagcccctttgacttcgatggtctccagcaagctgctgtaactcagcacttcttcatttaataacttggcttttccgagcatcgttgttttatcccgcagctccgcatgctgcctttctgattcattcaggttggcttccatactatccatccaaccggagaactgtcgaacgccatcctgataacttgtccacttggagagagctccttcgagttggcttttacaacgaatccctgcagacaaaagggatgcccacatatccttcacactctgcagctgctgctgaatagtgggaatgccttctggagaagtattctgaaggacagattctcccctggtcactatcattttcatctgaatctctttttcctgtttgactgataatagagcctcgagcttgagcgtcctgctgtccagcacacttttgtcggatgtcgggtggcagtatgaatccagcatgtgaatcgcatccgtcatccagtcttgtaattctttaatcccaagagagaactgattgtgttctgcaacgattctatccagtcttgacactttctcctttgttaaattgcttagcgctagatactgagaagacagctgcgacactctgtgcctaaagctcttgctggcagcttgtccttcccacagctgctgagctttctctttcagcctgttgagctgaggctcgtagcagtgtatttcctcaaggacagactggagcttctgctgctccctcctctttgctggcagatcatagaggcgattgctgctttcatggaccatcttctcagttttactcagccagtcctggataggctcagcacttacttcaaagtccttcatttggatctttagattctctagagcagattctttttggtggagatttgaatgaaaatttttccaatcttcttttgcagctgtaactttggcctggatccctttcgctttctctttggtcagcagggtactcagaagttcccctttagacagcatcatgtttagcttgtgctgtccattttcactttctgacaaaaactcctgtattttctgaagactagttgaaacttcacttatattttgaggtatatcaaaacacttggcggtagtgatttttgcattaaccaaccactgctggaaatccctgaaggcctttcgaaatctttgctgtaaaatctgttctttattctggcagcccttggatgcttgcaaacaaagacaattatactctttaatcaagccagaaacttttccactgtaggtactcaggtctctggaaaatcgacaaagttcattcagctgagacttgagatcctctgttctaggctctgctttttgcaaagcatccagtatctcttgtcctttgtgccagcattccactatctcctcatccgtgttcttgccttccaggagggttaactgctgagcccaggttttcagaagggcactgaactgttccagggcctgctccagttgagccacttggcctgagaattcctgctccgaaagggccatctggctgaccaggttctccaaacagctctgcgtttggaatacactgtcttcccactgcttccagtcggcacgcagggcctgcatctccgtgtgcatgagctcacacccactggcagttgtgttctgtttcacttcgggagccagcgactccactctgctgagacggcttgcaccaatctctctggaatctatcagctccttaatttttgataactttttctgggtggctgatgaatctccagacatatctgaccaccggtgaagttcttcctttgctgaatggagccaatctgtgaactcgtggaccgcatctaaatacattagatgatctttcacaatctcttccactttcctcattttttccttggcaacagtcattatatcattaaactgtgttttcagctcctcttgagctgtgtccttgaaagactcatcctctgtcttttcgtagagctccctggacttcgcaattagacggtgaagggctctcgtgtgatcttctgcctcagacaggatggactggaggtggtcaagcaggacgaacttctctttcagacctggctgtggttgtaagggatgttctattttttgatccactgattccatccactgctccaactggtttttcctctctacatagtcattccattggctaatcacagactctaaagtgctttgagcgtggacggaggagctcatgatgtcagcccacacttctttaagggtctctaactgagtctgaatcaccctctgaccttctttgttgctacttctcaaggcctgttcccccttgccaatggccatattcaacttaacttccccttcacctttcatcaggagaatatcctgtatttgtgacagccgtttctccagggtgtctttgctcccaagagtgctctctgcacaggccagtctgtcctgaatggccttcacccagaaccacatgctttgcagtgcttcctccagggcttcgtgctcctgaagggccacctggcagctccggagtttctctttggtcattctaagtaggttctggtggcttgtgaggagctgggaacacaggcggccctcctgcccagcaccgtggccttcttcactcagaagctgccctctctgggaaagcttatcaagagactctcttgcagccagcagttctcccaaaaacatttcaactttatgaacttcatttttcttctcaggaatgtgctgtttactctctcccaagttttccgtattgaacctttcttccatttcatggatccataagttcagttttctgtgctgatcttcaaagcttccaagttctgaagcacagtcttgaagagcctgcttatctttaaggcattgtttcagaaatgcttgaaactcttcattggcctttgtgatttgttcttgaatgctactgacaatttgtttagacaaatgtgcatacaaagtttgtccttcttgagtcactgcatcaagtttgctctgcccatcactgactgagtccaaaatgttctgaagatcatggagctttgcttctagaactttgctgtcaccggtgcgatctgatgattcttttgctgctgcctttgctcccaaaaaccattcttggaattcctgcatagactcactgaagtgtttttccagagattcctgcaggctggcctgggttttggagcacaactggctcacggcttcatgtttctttatcagaccagtcattgcacggcccaggctctccaactcagctgagtggtacttgcggcacaagctattgagattttcttgggtagagctgatgttgctttgttgactttgaagttctttttgtatatccttgacttttttcaatgcttcacaagtctcattttgggcacagttcatcaacgattcttccacttttgtgaaccatgttgttatgtcattaataaacttctccacttgtgtactttgagccgtgaaatccttcagggttccttttgctacttcagttatttctttggcatgctccagtttctgcattaagtctgcttctataaactgaaggtctggcggtgtttctagatttttagttaattctttcagatcattaactttggaatgcagttcttccaatctcaatgctttgtttttaacttcagactcaaattctttaagcagttcttcagctctgaggtggttatccaggttgctgatgttttctgccatctgtggaacgcagttgtttgaccatccctcaatctcatctctagttgacagtacatcatcccaaatggacaggcttactctcagcctatccatgttttcttcaagtttctctgatacatccagccatttgtccacggtgctctccatgtctgttttcaccaagctgaaatcactactgtgaattttcttcagctcagataacaagtgttttcctttgctggtaaagttatccaagtctttctgtttgtaattcattttgttcttggcagtttcatgcttggaaaaagcccatttaagatcctcctgatcttttatggtagttctggttacaatcacactgctggcattttctaagactttagatacagctgatttcaggttctgatattctctcattaagtcaataagtccacagcactgaccctgattttcatgaattagtcttttggtatcatcccaggtgacctctaagcggtttatctccctgtcaacttcaggtgcaaaagctacatctttctgggcaatttgcttggctttgtctttcaaccaacatagttcatgctcgtgagaattcaattcatcttctagctgattaaacactcttaacctctgctgaagagcttggcgggtaggttctttcaatcgctctttgtcagtcctttcttcaatgtcctcaatgcttttcagaagctcctctttctggtcttggaatgcttttttcaacactgccagagcatctgcctcactctgcttggttcccagaaggttctggatcctctctacctctccacagagctgatcagccgtggctctgcaggaagtcctttgctcagagctcccgattttcagatggtattgggctttggaaagaatgccatccagactgacggcagcagattctaatgctttagcattttgaagagcatcattgaggtccttttctatcaaatcagactcgttcttattcatactgttggttgcttccactgtttgcctcagctggcggagaatgccggacagagaggcatggctctggaggaattctgccaaatgggacagggcaagctgccgcctctccacaacctggctggcctcctcaaacagctggaagcagtcctcagcctttccctgcaggaggtggaggtcctcagcacggcccagagaacccaactttgctaagtgaccctgcagactctgcaattcgccctttttgctctctacttctgctgcgtggtccttatgccgagtaagggctacttgatggtccattatgctaatctcagaggtagtttgtaattcactgagaaacagtttaatccagacagaaaaggaaagcagcagctcatcaaattgctggtgttcagcaaccacagactgaagaaaattaatccttttgttaatgatctgtggtaaatctctccatctctcatccaactgctccaaatgtagtttcatcattttcacatcatctttggaggctactgagaacaatgattccttcaattgcaaaagtttgctatagaatgaggcctgggatacaacttcattttgcagtgcctgtattaactgaagttcaccttccactttgactctgtctgcagaaatgtccatttctggggaactggctttagcttcaccccgctctaaccaggtcaaaaaggatgatagttctttctctagcctctgccagtgggccagcagattctccagcgccgtctgtctctccttcgccctccttaggatgtcctcgtattgctgctgtagagccgcagcctcctgaacacaggaatctctgttcacaaccttcctggcactggctgagaaggcagtgatcgcgctgctcagtgactccagggcctggcagagatccatatgttcttgaagaactttgtatgtttctgtagctgaagaacatattttaattggaacagcaagtttatcttcaaattcagacacagattgctggatctttctaaggttctcttcaaacttttgctgctgagataaatgtcccaggattgttccttccagacactgtgcatgctctcgaagctcttccccgtatcttcttatttgtgtcaacttggctttaattcgagcagattctccagtggtaacaaactgagcaaaagactgggcttcttcttctaatcctacaatgctgctgagcttactttctatttcctgaattgtgaccttaatttggctgatttgcatgtccatggcagatgacgaagtttccaaggcattgagttctttttctttctcagttatccagacggacagagtctcaaaattactgccaaaatgatcccacttggttttcaccatttccatggttttaatatcttcttcaagcgtgtcttctaattttttgacttgttctttgattgacttggcctgctgttgaagcagctgcttattttggggcccaagcggtatctctgaagcttcctttacaaggttctcagcctggactgcaatactttctgtccgtttagaaaactcctttgtttgttccagttctgaagataaactttccaaactgctaaaactcaagaagcgttcatgactggaacctgtttgaaaaaggtatcttactactgtttctttgtttgtttcaaatcgctcccattttcttaatgtgacctggatgcggcgttcctgcctctcccggctgcgctccaggccatccagtgtgctctccagcttccgcagctcctcgtggcctcggtcaggcagccccccttctccctgctgcgcctgcgcgatctgctgctgcacatctctcttctttgctgagatccgctttgtcttttgctggtgatgaagaagtaactgctgtgcttcaaacagattttcagtatccaagatcttctcagcttgttcctggacttctttagagccagaaattaattcttcgagagaatttttgactatttctttgtactggacacagtccccaaaattgcttagcatcttttcaacctctgacagcagcgtcacaagagccttgaaagagctggataattttgccagctcatctccctgcttttgggcttcattctcagaagaaacttctgtcaaaactttcagcctggatttcagccagctgagggtctcaccccttttggtaacaccatttctgatctcttcaacggcacgtttaacctctccgtggttggcagtatcgatggcctcacccttgatcccctttaattgtgtctcatttgtagatatccaagatgagaactcagagaatctgctagtgtagtccttccacttgtctgggtcttccatgagcttcctgtaggtgctgtcaatggcagctctgagctctttgagagtcacgtgacaggttccaggtgtgtcccttactgggtcccgcactgggagtttcacacagagttcctcgatgagctgtaaccttttctcacagagatgatgaggacctttgtcactgaagaaaaccctgtgctctttaattatcttttcactgccttcctggggcatcagcttggtctctcgatccagctcagttctgcattcttctacagaggctaagaacctattcttctccacatcaatcttcagatgaagcaaatgataaggggcttctccttgaagatccttccattgtttgtggagctttcgaacagcttcctgcagcccctgctgctcctgctctggaaggatgtcggtgagttcatcacaagctttcaggaaagcattgagcaccctctgatccagctgactgaaaaactcagtgtgtctccgcaggagctcctctggatcccccttttcctccaggccctcctgagcaatccgcagtaccttctccaactctgctcgagactcctcaaacttcttcatcaagcgactgttggtttccacatgcttcttccaatctccagttttctttaccatactctgaaaagcaacatgaatatctgcaatctgtctttgtagcctcgtctgatcaaaatgctttaacacgttgctcaaggtcacaaacttttgaacactttgactgcctttctcaataagtgtcaaggttttcttacagttttcttgacaagctaacagttcctgatgtttttgtttaaaaagggcactcgattgtgcctcacgctcaagaactgtgataatttcattgattttcccaagtgagtcataaaaggacgtcatctgcttttctaattcctccaacggaatcaacagctgctgagactcataaaggagtggggagtaacattctttgaccttggttagctgctctttgagctttgacatggtcgcaaacatttcttttccttcttcttgggggctttctttggtaatgaggtgtgctgtctttgtaattatcttgtattgggcatccatcacaggcaccctctgctcaatatcctccaagtcttgaattaatagcttgacattcataaaagagacttctaagggttcagaaagtttcttatgggcttccgttgcaaaagcagacagggtaacaacacagtctgtgtattccttcttcattctgtccatctcatcagcttgagcatattgcttgacttccataaacaactccctccaccgcccatttagcaacagtaattgctgcttcaggtcacgggaaaccatctcatcacaggtttcaattagaaaattgccagcatcgttcatggcagtatgctgctgaatccaatgaggtaaatttcgaaaaaaatcctttttggcattttctgattgattgagcattttttcagcatcctctagccaggcttgcagactagccactgtattgccatagcgatcccagttagagatcacttcttccagcatgctcctcacactcctcacttctactgagagattcctccactgagcggtggtttcattcatgaatttcatcacattctcagcttcttccactgaaccatctgctttgacatacatctcagctgtctgtttcaagatctggtatgtcacctcatattgttcaaagaacttgctattttctataaaagacacgtagttttgtagaagctgctccactgactctctcctcccgtacttaatgatccaagacttcagctttgactctgcaagaaccagcagtgagagcagacggtactttaattctaaaaattccattttcattaggtgtagctctgatgtggaggaaacaaaatgaaacctctcggccatgtcctctaattgatcaggtggcactggaatcccgttaacagacctggtccggtagatttcatggaatgctcttttgtgggcatccgtgttttgaagcagatccttatgttgctcaagtttccgttgtatcgtgtttgctgtttcctcgtggacctgttgaacggttatttcctctctcagggccacctccgctctgtacagccaggcacctatggtgcccagaggtgcaggaagagatttatcaagctgtatatgccagtcaaagagcctggaggtcactctatcccaagattgttttaccaatgcttggtcaagtgacaatttaccgtctctgtgtaatggttgtattaaatgttcaatctgtttcctcttcatttcatattgaactctgaagtgcttaaatgactgatatttatcctgtaaatttgattccaccatctgtgctcttgtcaaatctctctcaaattgttctatccaaactttcatttccttaaaaattactctgtcttctctatcatcctcttgcccatcagtgcttgcattgtggatgtcaggataatgtttcagaaactgggctacataggtcataatagatttctcatctggtttatccacatcaacgtcttcaggatctagcagtcttgggatccccagttctgtttcggcgatagtgaaagcatcctccaaattttctcggttggatctgcctttcactgtctccaagtccaccaattccggtcgaatggcatgaataactgaatgaaaggcaaccccgcttctccaactcttcccaaaatcttttacttctattccagtctgcttgccagctgtgtactgaacccactttaataaagccttcttagcatttccttggatcttggtggtcaccttccgtttacttggtgggctgggagtctcagagctaactatgctgtccacggaggatgcgctgctggacaaagactggagctggggcaggttgctggtcaactcttcaatctggaaatatagaataatggtccacatcaatccaagaactattgagggtcggccatcagctatatcggtggagttaatgttgactaatttaatctttcttccttcgaggaacttgagtgccgtgccaatgttagccacagcatggattcgcttcatccggcgtccttgttcacaaggcagtttctgcccagacaggacctccagaagggcaagcagtttaacaccatctttcatgtcttcaaaaagatcgtccaccaccattggaggtttccgcttggccagatgagagttgatccattttgtgaaagttcgtttttgtactatctcttgctcatcttgcagcctctgcatcacattggcgatatcccgaggacaccgggaggcccctctggaggttgccatggtccctccggaagcacgaagccaacaccaagagactcttcactggaggcagcacagggctacaccactctagaaaacatgcttggacttttctagatctattctgtcataaatgaattccaggcctttgcagcactcaacaaggaggcagctctcccaaagactgaactgcttctttttcttcttccgttttaagactgtcctcttacatgaactcaagaaccttctctctcggcctcgttcagtttcccagcagcaaggcgaagcgagcgaacgcttcctcccggctctctgcgcccaggctcggcgggaccccggggatgcgcggctgtccgcccgccctgtcgccgggatcgggcgcggtctgcaggactgcgggagcccagccgccctggtgacagaggacaacaatctcagcccgctgcggccggcggccgcggcccggcgcccgcgctcaccctggctggctcgcccacact

SEQ ID NO: 9570 - RNA, 14163 nt, Homo sapiens
  source 1..14163: mol_type = other RNA
agttcttcagtggcaagctttatcaaaatcttccttaaaatgcttcctagaaaccaaattcttctctagttcttgtaaccggtgactgcacttttgtaaaacactgtcatagacactctgcaattcctgaagcttccccagcacttcactcttttcctgctctgtgacttccttcattagttcgcgaccctgggcccaaagtccagtgacttcattttggtaagtcttgaggctggcttgtgcactcttacatgttttgacttgtttgctcacatcatctggtaacagacagatgtgttcacggaacattatctttcgctcatgttgctgaatttggctggtggcctggaacactgccatgagaaactgggttttctcggacaaggctttgtttaagtactttcttcgctggcccactaagtcactgagacaattcacgtggctttgtgcatcagagagagccttctggatgacctgtcgctcattgagaccaagatctgccatgaccctgtctgcgtcctttataagcgatttcaggagcatctgcttggcctccagttcactgcagatggccaggtgatccatgagaaggttctgagccatatctggaggagggctctgcttaagggcctcggcgatgttgggttgttgctcttctgcccactccattagctcctgaaatctggactgcaccacatttaactcctccaagttggtgactgacacttggattttccttttaatgaggtcctcaagctgaaaccaacgttgctctaaatgactcgtctgttctttgactaactccttgtcatctaaattcagatgctctatcattttctgcttttgatctttcagatcttcaatagcatactttctctcctgcaatgccaatgctaactttttcaaagcttccaggtggacagctgtactctctgcatcagatctggccaagttatcccattctgtagtaaatttttctaggaacacttcaacaacattcatacagtcatggtaatctcttgttctctgaagatcctcttccctttgcaagcacaggttgttagactgacggcacaaatcgagccactgatcatttaaatgatttatttccttgtgttcaggcgattcctccttctttgttaacttattcaccttttctattatggtgttcacggatgcctgtttgctctgtagtttcttaacaaaatccttaacttgtgaaaccatgttctgtgcaatgttcagctccagctcagagtgcctcctcttcatgttctgcagttgctgatcagcatcttgcaggtaaatccagagctcagacttcaggtgcttgatctcttcccagccctgagttaagttctgggcctggacaagcttttgttcaatcgtttgctctgtttgttgaatgtcttttgctgtggttttcaccgaagcatttgacaggtcacacatggagcaaaggagatctaggtaggtccttgcctgctcttgcaaagctctgaagtgtttgacctgcttaatggcttctgccctactaagaggtggttgaggacttggctctaaatccggctggactgcagaaagccaggcctggcactgctgcagggtgtcttgtcggctgacgtgcttctgaagttcgtgttccaaactctggtacatcctctgagctgtgctgcagatcgctgagtagctgtcctttgtgccctgcagatgagcatgcacgttttgtttaagtttcgcttgcaggtggtctgcacattggccaatcaaagtatcacctttcatttgaagattgttcaaacggtcttcaaaaccagcaatttcttccatcattgccttgtggtgggccaattgctgggtgattgtctccaggctgcttgtctccaggaggtcaggtgccaccagtctgccagacatctgcagcagccacttttcgacctcttggagctcactgttgtagtcttcatggtctttgactttcgcctccagactgaagacatgctcctttcctatgctgcacaggtcctggtaatcactttgaagttgatctattttgtcctttaaagtgacgtcctgcaccagttccaaaagagcttcacccttctctctcactgactttactgatggttcatgggacagcaccgtttgttgaagtgacttgtatttagataactgagcttttttctcatataattccattttgggttcttcaggaacatgtagaatttcctggtattctgctatccactgtgtcagtgctttgcatttatctgagaattcctttgctaaatgaagacctttttccagcgtcatgtgttctttccggacagtgctggtcagttccttcaactgctccatgtgatcatgaatctcctttcttaacctctctgcctcgccttcctccaagtatttaacagccctctctcctttctcccgggctgatttcagcaaactgtgacctttctccatgtctttgagcaaaacctccaacgtcttcaatttcttccccatcattactgtatctactttgtcaatcttggtagccacattcttgaagtttttatgagtagagccataccaatcagaataggaactgagggatgattctgattcctccaaactctgaatctcctcctccaggaattttatttgttccagcacttggagaagcagggcctggtatctggaagtcagctgggtggcctggcaacccattctgctgttcacgtggctctcgtccagtatctcctgagctctagctcccacttcctcaacttcatctctgtatgcagtcacttcttcgtgccacttcttcatctgatgtaattgtatctccttggttgccctgttagactgacgtctggtcctgggactaactttctcctctgctgttttgagccattcatctacttgctgaaacttttgctccattagcctcaatttgttcaccacgttattgaactgagttcgagtctcggacagcctgtgctggtaagcctgccagtcttgccggagagactctaaagcccggtcctctgcctgtgggatacctgatgggatcacatcctctctggtgtgcagcactgagttcaacagggcctgcccctctgcacagtgtacctgtagctcctgaagatcacgcaatgttgtctcatgagtgtgggcatcaccttcaagaactgaatactggtcgagcttttcttgttcttgccccaaccaaacttcaaatgcctttaggtctctctgatactcttggtgcaggcggacaagtttttcagacttggttacggcttccttggccctctcttggatggctctgtatcgttcctgtagatcctggagttctagctgggtgacatagtgttctgtcatgccagcccctttgacttcgatggtctccagcaagctgctgtaactcagcacttcttcatttaataacttggcttttccgagcatcgttgttttatcccgcagctccgcatgctgcctttctgattcattcaggttggcttccatactatccatccaaccggagaactgtcgaacgccatcctgataacttgtccacttggagagagctccttcgagttggcttttacaacgaatccctgcagacaaaagggatgcccacatatccttcacactctgcagctgctgctgaatagtgggaatgccttctggagaagtattctgaaggacagattctcccctggtcactatcattttcatctgaatctctttttcctgtttgactgataatagagcctcgagcttgagcgtcctgctgtccagcacacttttgtcggatgtcgggtggcagtatgaatccagcatgtgaatcgcatccgtcatccagtcttgtaattctttaatcccaagagagaactgattgtgttctgcaacgattctatccagtcttgacactttctcctttgttaaattgcttagcgctagatactgagaagacagctgcgacactctgtgcctaaagctcttgctggcagcttgtccttcccacagctgctgagctttctctttcagcctgttgagctgaggctcgtagcagtgtatttcctcaaggacagactggagcttctgctgctccctcctctttgctggcagatcatagaggcgattgctgctttcatggaccatcttctcagttttactcagccagtcctggataggctcagcacttacttcaaagtccttcatttggatctttagattctctagagcagattctttttggtggagatttgaatgaaaatttttccaatcttcttttgcagctgtaactttggcctggatccctttcgctttctctttggtcagcagggtactcagaagttcccctttagacagcatcatgtttagcttgtgctgtccattttcactttctgacaaaaactcctgtattttctgaagactagttgaaacttcacttatattttgaggtatatcaaaacacttggcggtagtgatttttgcattaaccaaccactgctggaaatccctgaaggcctttcgaaatctttgctgtaaaatctgttctttattctggcagcccttggatgcttgcaaacaaagacaattatactctttaatcaagccagaaacttttccactgtaggtactcaggtctctggaaaatcgacaaagttcattcagctgagacttgagatcctctgttctaggctctgctttttgcaaagcatccagtatctcttgtcctttgtgccagcattccactatctcctcatccgtgttcttgccttccaggagggttaactgctgagcccaggttttcagaagggcactgaactgttccagggcctgctccagttgagccacttggcctgagaattcctgctccgaaagggccatctggctgaccaggttctccaaacagctctgcgtttggaatacactgtcttcccactgcttccagtcggcacgcagggcctgcatctccgtgtgcatgagctcacacccactggcagttgtgttctgtttcacttcgggagccagcgactccactctgctgagacggcttgcaccaatctctctggaatctatcagctccttaatttttgataactttttctgggtggctgatgaatctccagacatatctgaccaccggtgaagttcttcctttgctgaatggagccaatctgtgaactcgtggaccgcatctaaatacattagatgatctttcacaatctcttccactttcctcattttttccttggcaacagtcattatatcattaaactgtgttttcagctcctcttgagctgtgtccttgaaagactcatcctctgtcttttcgtagagctccctggacttcgcaattagacggtgaagggctctcgtgtgatcttctgcctcagacaggatggactggaggtggtcaagcaggacgaacttctctttcagacctggctgtggttgtaagggatgttctattttttgatccactgattccatccactgctccaactggtttttcctctctacatagtcattccattggctaatcacagactctaaagtgctttgagcgtggacggaggagctcatgatgtcagcccacacttctttaagggtctctaactgagtctgaatcaccctctgaccttctttgttgctacttctcaaggcctgttcccccttgccaatggccatattcaacttaacttccccttcacctttcatcaggagaatatcctgtatttgtgacagccgtttctccagggtgtctttgctcccaagagtgctctctgcacaggccagtctgtcctgaatggccttcacccagaaccacatgctttgcagtgcttcctccagggcttcgtgctcctgaagggccacctggcagctccggagtttctctttggtcattctaagtaggttctggtggcttgtgaggagctgggaacacaggcggccctcctgcccagcaccgtggccttcttcactcagaagctgccctctctgggaaagcttatcaagagactctcttgcagccagcagttctcccaaaaacatttcaactttatgaacttcatttttcttctcaggaatgtgctgtttactctctcccaagttttccgtattgaacctttcttccatttcatggatccataagttcagttttctgtgctgatcttcaaagcttccaagttctgaagcacagtcttgaagagcctgcttatctttaaggcattgtttcagaaatgcttgaaactcttcattggcctttgtgatttgttcttgaatgctactgacaatttgtttagacaaatgtgcatacaaagtttgtccttcttgagtcactgcatcaagtttgctctgcccatcactgactgagtccaaaatgttctgaagatcatggagctttgcttctagaactttgctgtcaccggtgcgatctgatgattcttttgctgctgcctttgctcccaaaaaccattcttggaattcctgcatagactcactgaagtgtttttccagagattcctgcaggctggcctgggttttggagcacaactggctcacggcttcatgtttctttatcagaccagtcattgcacggcccaggctctccaactcagctgagtggtacttgcggcacaagctattgagattttcttgggtagagctgatgttgctttgttgactttgaagttctttttgtatatccttgacttttttcaatgcttcacaagtctcattttgggcacagttcatcaacgattcttccacttttgtgaaccatgttgttatgtcattaataaacttctccacttgtgtactttgagccgtgaaatccttcagggttccttttgctacttcagttatttctttggcatgctccagtttctgcattaagtctgcttctataaactgaaggtctggcggtgtttctagatttttagttaattctttcagatcattaactttggaatgcagttcttccaatctcaatgctttgtttttaacttcagactcaaattctttaagcagttcttcagctctgaggtggttatccaggttgctgatgttttctgccatctgtggaacgcagttgtttgaccatccctcaatctcatctctagttgacagtacatcatcccaaatggacaggcttactctcagcctatccatgttttcttcaagtttctctgatacatccagccatttgtccacggtgctctccatgtctgttttcaccaagctgaaatcactactgtgaattttcttcagctcagataacaagtgttttcctttgctggtaaagttatccaagtctttctgtttgtaattcattttgttcttggcagtttcatgcttggaaaaagcccatttaagatcctcctgatcttttatggtagttctggttacaatcacactgctggcattttctaagactttagatacagctgatttcaggttctgatattctctcattaagtcaataagtccacagcactgaccctgattttcatgaattagtcttttggtatcatcccaggtgacctctaagcggtttatctccctgtcaacttcaggtgcaaaagctacatctttctgggcaatttgcttggctttgtctttcaaccaacatagttcatgctcgtgagaattcaattcatcttctagctgattaaacactcttaacctctgctgaagagcttggcgggtaggttctttcaatcgctctttgtcagtcctttcttcaatgtcctcaatgcttttcagaagctcctctttctggtcttggaatgcttttttcaacactgccagagcatctgcctcactctgcttggttcccagaaggttctggatcctctctacctctccacagagctgatcagccgtggctctgcaggaagtcctttgctcagagctcccgattttcagatggtattgggctttggaaagaatgccatccagactgacggcagcagattctaatgctttagcattttgaagagcatcattgaggtccttttctatcaaatcagactcgttcttattcatactgttggttgcttccactgtttgcctcagctggcggagaatgccggacagagaggcatggctctggaggaattctgccaaatgggacagggcaagctgccgcctctccacaacctggctggcctcctcaaacagctggaagcagtcctcagcctttccctgcaggaggtggaggtcctcagcacggcccagagaacccaactttgctaagtgaccctgcagactctgcaattcgccctttttgctctctacttctgctgcgtggtccttatgccgagtaagggctacttgatggtccattatgctaatctcagaggtagtttgtaattcactgagaaacagtttaatccagacagaaaaggaaagcagcagctcatcaaattgctggtgttcagcaaccacagactgaagaaaattaatccttttgttaatgatctgtggtaaatctctccatctctcatccaactgctccaaatgtagtttcatcattttcacatcatctttggaggctactgagaacaatgattccttcaattgcaaaagtttgctatagaatgaggcctgggatacaacttcattttgcagtgcctgtattaactgaagttcaccttccactttgactctgtctgcagaaatgtccatttctggggaactggctttagcttcaccccgctctaaccaggtcaaaaaggatgatagttctttctctagcctctgccagtgggccagcagattctccagcgccgtctgtctctccttcgccctccttaggatgtcctcgtattgctgctgtagagccgcagcctcctgaacacaggaatctctgttcacaaccttcctggcactggctgagaaggcagtgatcgcgctgctcagtgactccagggcctggcagagatccatatgttcttgaagaactttgtatgtttctgtagctgaagaacatattttaattggaacagcaagtttatcttcaaattcagacacagattgctggatctttctaaggttctcttcaaacttttgctgctgagataaatgtcccaggattgttccttccagacactgtgcatgctctcgaagctcttccccgtatcttcttatttgtgtcaacttggctttaattcgagcagattctccagtggtaacaaactgagcaaaagactgggcttcttcttctaatcctacaatgctgctgagcttactttctatttcctgaattgtgaccttaatttggctgatttgcatgtccatggcagatgacgaagtttccaaggcattgagttctttttctttctcagttatccagacggacagagtctcaaaattactgccaaaatgatcccacttggttttcaccatttccatggttttaatatcttcttcaagcgtgtcttctaattttttgacttgttctttgattgacttggcctgctgttgaagcagctgcttattttggggcccaagcggtatctctgaagcttcctttacaaggttctcagcctggactgcaatactttctgtccgtttagaaaactcctttgtttgttccagttctgaagataaactttccaaactgctaaaactcaagaagcgttcatgactggaacctgtttgaaaaaggtatcttactactgtttctttgtttgtttcaaatcgctcccattttcttaatgtgacctggatgcggcgttcctgcctctcccggctgcgctccaggccatccagtgtgctctccagcttccgcagctcctcgtggcctcggtcaggcagccccccttctccctgctgcgcctgcgcgatctgctgctgcacatctctcttctttgctgagatccgctttgtcttttgctggtgatgaagaagtaactgctgtgcttcaaacagattttcagtatccaagatcttctcagcttgttcctggacttctttagagccagaaattaattcttcgagagaatttttgactatttctttgtactggacacagtccccaaaattgcttagcatcttttcaacctctgacagcagcgtcacaagagccttgaaagagctggataattttgccagctcatctccctgcttttgggcttcattctcagaagaaacttctgtcaaaactttcagcctggatttcagccagctgagggtctcaccccttttggtaacaccatttctgatctcttcaacggcacgtttaacctctccgtggttggcagtatcgatggcctcacccttgatcccctttaattgtgtctcatttgtagatatccaagatgagaactcagagaatctgctagtgtagtccttccacttgtctgggtcttccatgagcttcctgtaggtgctgtcaatggcagctctgagctctttgagagtcacgtgacaggttccaggtgtgtcccttactgggtcccgcactgggagtttcacacagagttcctcgatgagctgtaaccttttctcacagagatgatgaggacctttgtcactgaagaaaaccctgtgctctttaattatcttttcactgccttcctggggcatcagcttggtctctcgatccagctcagttctgcattcttctacagaggctaagaacctattcttctccacatcaatcttcagatgaagcaaatgataaggggcttctccttgaagatccttccattgtttgtggagctttcgaacagcttcctgcagcccctgctgctcctgctctggaaggatgtcggtgagttcatcacaagctttcaggaaagcattgagcaccctctgatccagctgactgaaaaactcagtgtgtctccgcaggagctcctctggatcccccttttcctccaggccctcctgagcaatccgcagtaccttctccaactctgctcgagactcctcaaacttcttcatcaagcgactgttggtttccacatgcttcttccaatctccagttttctttaccatactctgaaaagcaacatgaatatctgcaatctgtctttgtagcctcgtctgatcaaaatgctttaacacgttgctcaaggtcacaaacttttgaacactttgactgcctttctcaataagtgtcaaggttttcttacagttttcttgacaagctaacagttcctgatgtttttgtttaaaaagggcactcgattgtgcctcacgctcaagaactgtgataatttcattgattttcccaagtgagtcataaaaggacgtcatctgcttttctaattcctccaacggaatcaacagctgctgagactcataaaggagtggggagtaacattctttgaccttggttagctgctctttgagctttgacatggtcgcaaacatttcttttccttcttcttgggggctttctttggtaatgaggtgtgctgtctttgtaattatcttgtattgggcatccatcacaggcaccctctgctcaatatcctccaagtcttgaattaatagcttgacattcataaaagagacttctaagggttcagaaagtttcttatgggcttccgttgcaaaagcagacagggtaacaacacagtctgtgtattccttcttcattctgtccatctcatcagcttgagcatattgcttgacttccataaacaactccctccaccgcccatttagcaacagtaattgctgcttcaggtcacgggaaaccatctcatcacaggtttcaattagaaaattgccagcatcgttcatggcagtatgctgctgaatccaatgaggtaaatttcgaaaaaaatcctttttggcattttctgattgattgagcattttttcagcatcctctagccaggcttgcagactagccactgtattgccatagcgatcccagttagagatcacttcttccagcatgctcctcacactcctcacttctactgagagattcctccactgagcggtggtttcattcatgaatttcatcacattctcagcttcttccactgaaccatctgctttgacatacatctcagctgtctgtttcaagatctggtatgtcacctcatattgttcaaagaacttgctattttctataaaagacacgtagttttgtagaagctgctccactgactctctcctcccgtacttaatgatccaagacttcagctttgactctgcaagaaccagcagtgagagcagacggtactttaattctaaaaattccattttcattaggtgtagctctgatgtggaggaaacaaaatgaaacctctcggccatgtcctctaattgatcaggtggcactggaatcccgttaacagacctggtccggtagatttcatggaatgctcttttgtgggcatccgtgttttgaagcagatccttatgttgctcaagtttccgttgtatcgtgtttgctgtttcctcgtggacctgttgaacggttatttcctctctcagggccacctccgctctgtacagccaggcacctatggtgcccagaggtgcaggaagagatttatcaagctgtatatgccagtcaaagagcctggaggtcactctatcccaagattgttttaccaatgcttggtcaagtgacaatttaccgtctctgtgtaatggttgtattaaatgttcaatctgtttcctcttcatttcatattgaactctgaagtgcttaaatgactgatatttatcctgtaaatttgattccaccatctgtgctcttgtcaaatctctctcaaattgttctatccaaactttcatttccttaaaaattactctgtcttctctcttaaaattttgtacagaatttgcaaaagatgggaaacctggaagtatttcatcatcctcttgcccatcagtgcttgcattgtggatgtcaggataatgtttcagaaactgggctacataggtcataatagatttctcatctggtttatccacatcaacgtcttcaggatctagcagtcttgggatccccagttctgtttcggcgatagtgaaagcatcctccaaattttctcggttggatctgcctttcactgtctccaagtccaccaattccggtcgaatggcatgaataactgaatgaaaggcaaccccgcttctccaactcttcccaaaatcttttacttctattccagtctgcttgccagctgtgtactgaacccactttaataaagccttcttagcatttccttggatcttggtggtcaccttccgtttacttggtgggctgggagtctcagagctaactatgctgtccacggaggatgcgctgctggacaaagactggagctggggcaggttgctggtcaactcttcaatctggaaatatagaataatggtccacatcaatccaagaactattgagggtcggccatcagctatatcggtggagttaatgttgactaatttaatcggtgatcctctgtgcatggactttcttccttcgaggaacttgagtgccgtgccaatgttagccacagcatggattcgcttcatccggcgtccttgttcacaaggcagtttctgcccagacaggacctccagaagggcaagcagtttaacaccatctttcatgtcttcaaaaagatcgtccaccaccattggaggtttccgcttggccagatgagagttgatccattttgtgaaagttcgtttttgtactatctcttgctcatcttgcagcctctgcatcacattggcgatatcccgaggacaccgggaggcccctctggaggttgccatggtccctccggaagcacgaagccaacaccaagagactcttcactggaggcagcacagggctacaccactctagaaaacatgcttggacttttctagatctattctgtcataaatgaattccaggcctttgcagcactcaacaaggaggcagctctcccaaagactgaactgcttctttttcttcttccgttttaagactgtcctcttacatgaactcaagaacctcctggagatgcacggccttgggcgtttctccgcagctgcaaagctgtgctgtgacccacccgctcagcgagcctttataccgggaccacctcccgggggtcgaggtgggaaggaaatgtccctgagagccgggacgcgctgcctccgctgcctggaggagctgcgctgtcctgccagcta

SEQ ID NO: 9571 - RNA, 14356 nt, Homo sapiens
  source 1..14356: mol_type = other RNA
agttcttcagtggcaagctttatcaaaatcttccttaaaatgcttcctagaaaccaaattcttctctagttcttgtaaccggtgactgcacttttgtaaaacactgtcatagacactctgcaattcctgaagcttccccagcacttcactcttttcctgctctgtgacttccttcattagttcgcgaccctgggcccaaagtccagtgacttcattttggtaagtcttgaggctggcttgtgcactcttacatgttttgacttgtttgctcacatcatctggtaacagacagatgtgttcacggaacattatctttcgctcatgttgctgaatttggctggtggcctggaacactgccatgagaaactgggttttctcggacaaggctttgtttaagtactttcttcgctggcccactaagtcactgagacaattcacgtggctttgtgcatcagagagagccttctggatgacctgtcgctcattgagaccaagatctgccatgaccctgtctgcgtcctttataagcgatttcaggagcatctgcttggcctccagttcactgcagatggccaggtgatccatgagaaggttctgagccatatctggaggagggctctgcttaagggcctcggcgatgttgggttgttgctcttctgcccactccattagctcctgaaatctggactgcaccacatttaactcctccaagttggtgactgacacttggattttccttttaatgaggtcctcaagctgaaaccaacgttgctctaaatgactcgtctgttctttgactaactccttgtcatctaaattcagatgctctatcattttctgcttttgatctttcagatcttcaatagcatactttctctcctgcaatgccaatgctaactttttcaaagcttccaggtggacagctgtactctctgcatcagatctggccaagttatcccattctgtagtaaatttttctaggaacacttcaacaacattcatacagtcatggtaatctcttgttctctgaagatcctcttccctttgcaagcacaggttgttagactgacggcacaaatcgagccactgatcatttaaatgatttatttccttgtgttcaggcgattcctccttctttgttaacttattcaccttttctattatggtgttcacggatgcctgtttgctctgtagtttcttaacaaaatccttaacttgtgaaaccatgttctgtgcaatgttcagctccagctcagagtgcctcctcttcatgttctgcagttgctgatcagcatcttgcaggtaaatccagagctcagacttcaggtgcttgatctcttcccagccctgagttaagttctgggcctggacaagcttttgttcaatcgtttgctctgtttgttgaatgtcttttgctgtggttttcaccgaagcatttgacaggtcacacatggagcaaaggagatctaggtaggtccttgcctgctcttgcaaagctctgaagtgtttgacctgcttaatggcttctgccctactaagaggtggttgaggacttggctctaaatccggctggactgcagaaagccaggcctggcactgctgcagggtgtcttgtcggctgacgtgcttctgaagttcgtgttccaaactctggtacatcctctgagctgtgctgcagatcgctgagtagctgtcctttgtgccctgcagatgagcatgcacgttttgtttaagtttcgcttgcaggtggtctgcacattggccaatcaaagtatcacctttcatttgaagattgttcaaacggtcttcaaaaccagcaatttcttccatcattgccttgtggtgggccaattgctgggtgattgtctccaggctgcttgtctccaggaggtcaggtgccaccagtctgccagacatctgcagcagccacttttcgacctcttggagctcactgttgtagtcttcatggtctttgactttcgcctccagactgaagacatgctcctttcctatgctgcacaggtcctggtaatcactttgaagttgatctattttgtcctttaaagtgacgtcctgcaccagttccaaaagagcttcacccttctctctcactgactttactgatggttcatgggacagcaccgtttgttgaagtgacttgtatttagataactgagcttttttctcatataattccattttgggttcttcaggaacatgtagaatttcctggtattctgctatccactgtgtcagtgctttgcatttatctgagaattcctttgctaaatgaagacctttttccagcgtcatgtgttctttccggacagtgctggtcagttccttcaactgctccatgtgatcatgaatctcctttcttaacctctctgcctcgccttcctccaagtatttaacagccctctctcctttctcccgggctgatttcagcaaactgtgacctttctccatgtctttgagcaaaacctccaacgtcttcaatttcttccccatcattactgtatctactttgtcaatcttggtagccacattcttgaagtttttatgagtagagccataccaatcagaataggaactgagggatgattctgattcctccaaactctgaatctcctcctccaggaattttatttgttccagcacttggagaagcagggcctggtatctggaagtcagctgggtggcctggcaacccattctgctgttcacgtggctctcgtccagtatctcctgagctctagctcccacttcctcaacttcatctctgtatgcagtcacttcttcgtgccacttcttcatctgatgtaattgtatctccttggttgccctgttagactgacgtctggtcctgggactaactttctcctctgctgttttgagccattcatctacttgctgaaacttttgctccattagcctcaatttgttcaccacgttattgaactgagttcgagtctcggacagcctgtgctggtaagcctgccagtcttgccggagagactctaaagcccggtcctctgcctgtgggatacctgatgggatcacatcctctctggtgtgcagcactgagttcaacagggcctgcccctctgcacagtgtacctgtagctcctgaagatcacgcaatgttgtctcatgagtgtgggcatcaccttcaagaactgaatactggtcgagcttttcttgttcttgccccaaccaaacttcaaatgcctttaggtctctctgatactcttggtgcaggcggacaagtttttcagacttggttacggcttccttggccctctcttggatggctctgtatcgttcctgtagatcctggagttctagctgggtgacatagtgttctgtcatgccagcccctttgacttcgatggtctccagcaagctgctgtaactcagcacttcttcatttaataacttggcttttccgagcatcgttgttttatcccgcagctccgcatgctgcctttctgattcattcaggttggcttccatactatccatccaaccggagaactgtcgaacgccatcctgataacttgtccacttggagagagctccttcgagttggcttttacaacgaatccctgcagacaaaagggatgcccacatatccttcacactctgcagctgctgctgaatagtgggaatgccttctggagaagtattctgaaggacagattctcccctggtcactatcattttcatctgaatctctttttcctgtttgactgataatagagcctcgagcttgagcgtcctgctgtccagcacacttttgtcggatgtcgggtggcagtatgaatccagcatgtgaatcgcatccgtcatccagtcttgtaattctttaatcccaagagagaactgattgtgttctgcaacgattctatccagtcttgacactttctcctttgttaaattgcttagcgctagatactgagaagacagctgcgacactctgtgcctaaagctcttgctggcagcttgtccttcccacagctgctgagctttctctttcagcctgttgagctgaggctcgtagcagtgtatttcctcaaggacagactggagcttctgctgctccctcctctttgctggcagatcatagaggcgattgctgctttcatggaccatcttctcagttttactcagccagtcctggataggctcagcacttacttcaaagtccttcatttggatctttagattctctagagcagattctttttggtggagatttgaatgaaaatttttccaatcttcttttgcagctgtaactttggcctggatccctttcgctttctctttggtcagcagggtactcagaagttcccctttagacagcatcatgtttagcttgtgctgtccattttcactttctgacaaaaactcctgtattttctgaagactagttgaaacttcacttatattttgaggtatatcaaaacacttggcggtagtgatttttgcattaaccaaccactgctggaaatccctgaaggcctttcgaaatctttgctgtaaaatctgttctttattctggcagcccttggatgcttgcaaacaaagacaattatactctttaatcaagccagaaacttttccactgtaggtactcaggtctctggaaaatcgacaaagttcattcagctgagacttgagatcctctgttctaggctctgctttttgcaaagcatccagtatctcttgtcctttgtgccagcattccactatctcctcatccgtgttcttgccttccaggagggttaactgctgagcccaggttttcagaagggcactgaactgttccagggcctgctccagttgagccacttggcctgagaattcctgctccgaaagggccatctggctgaccaggttctccaaacagctctgcgtttggaatacactgtcttcccactgcttccagtcggcacgcagggcctgcatctccgtgtgcatgagctcacacccactggcagttgtgttctgtttcacttcgggagccagcgactccactctgctgagacggcttgcaccaatctctctggaatctatcagctccttaatttttgataactttttctgggtggctgatgaatctccagacatatctgaccaccggtgaagttcttcctttgctgaatggagccaatctgtgaactcgtggaccgcatctaaatacattagatgatctttcacaatctcttccactttcctcattttttccttggcaacagtcattatatcattaaactgtgttttcagctcctcttgagctgtgtccttgaaagactcatcctctgtcttttcgtagagctccctggacttcgcaattagacggtgaagggctctcgtgtgatcttctgcctcagacaggatggactggaggtggtcaagcaggacgaacttctctttcagacctggctgtggttgtaagggatgttctattttttgatccactgattccatccactgctccaactggtttttcctctctacatagtcattccattggctaatcacagactctaaagtgctttgagcgtggacggaggagctcatgatgtcagcccacacttctttaagggtctctaactgagtctgaatcaccctctgaccttctttgttgctacttctcaaggcctgttcccccttgccaatggccatattcaacttaacttccccttcacctttcatcaggagaatatcctgtatttgtgacagccgtttctccagggtgtctttgctcccaagagtgctctctgcacaggccagtctgtcctgaatggccttcacccagaaccacatgctttgcagtgcttcctccagggcttcgtgctcctgaagggccacctggcagctccggagtttctctttggtcattctaagtaggttctggtggcttgtgaggagctgggaacacaggcggccctcctgcccagcaccgtggccttcttcactcagaagctgccctctctgggaaagcttatcaagagactctcttgcagccagcagttctcccaaaaacatttcaactttatgaacttcatttttcttctcaggaatgtgctgtttactctctcccaagttttccgtattgaacctttcttccatttcatggatccataagttcagttttctgtgctgatcttcaaagcttccaagttctgaagcacagtcttgaagagcctgcttatctttaaggcattgtttcagaaatgcttgaaactcttcattggcctttgtgatttgttcttgaatgctactgacaatttgtttagacaaatgtgcatacaaagtttgtccttcttgagtcactgcatcaagtttgctctgcccatcactgactgagtccaaaatgttctgaagatcatggagctttgcttctagaactttgctgtcaccggtgcgatctgatgattcttttgctgctgcctttgctcccaaaaaccattcttggaattcctgcatagactcactgaagtgtttttccagagattcctgcaggctggcctgggttttggagcacaactggctcacggcttcatgtttctttatcagaccagtcattgcacggcccaggctctccaactcagctgagtggtacttgcggcacaagctattgagattttcttgggtagagctgatgttgctttgttgactttgaagttctttttgtatatccttgacttttttcaatgcttcacaagtctcattttgggcacagttcatcaacgattcttccacttttgtgaaccatgttgttatgtcattaataaacttctccacttgtgtactttgagccgtgaaatccttcagggttccttttgctacttcagttatttctttggcatgctccagtttctgcattaagtctgcttctataaactgaaggtctggcggtgtttctagatttttagttaattctttcagatcattaactttggaatgcagttcttccaatctcaatgctttgtttttaacttcagactcaaattctttaagcagttcttcagctctgaggtggttatccaggttgctgatgttttctgccatctgtggaacgcagttgtttgaccatccctcaatctcatctctagttgacagtacatcatcccaaatggacaggcttactctcagcctatccatgttttcttcaagtttctctgatacatccagccatttgtccacggtgctctccatgtctgttttcaccaagctgaaatcactactgtgaattttcttcagctcagataacaagtgttttcctttgctggtaaagttatccaagtctttctgtttgtaattcattttgttcttggcagtttcatgcttggaaaaagcccatttaagatcctcctgatcttttatggtagttctggttacaatcacactgctggcattttctaagactttagatacagctgatttcaggttctgatattctctcattaagtcaataagtccacagcactgaccctgattttcatgaattagtcttttggtatcatcccaggtgacctctaagcggtttatctccctgtcaacttcaggtgcaaaagctacatctttctgggcaatttgcttggctttgtctttcaaccaacatagttcatgctcgtgagaattcaattcatcttctagctgattaaacactcttaacctctgctgaagagcttggcgggtaggttctttcaatcgctctttgtcagtcctttcttcaatgtcctcaatgcttttcagaagctcctctttctggtcttggaatgcttttttcaacactgccagagcatctgcctcactctgcttggttcccagaaggttctggatcctctctacctctccacagagctgatcagccgtggctctgcaggaagtcctttgctcagagctcccgattttcagatggtattgggctttggaaagaatgccatccagactgacggcagcagattctaatgctttagcattttgaagagcatcattgaggtccttttctatcaaatcagactcgttcttattcatactgttggttgcttccactgtttgcctcagctggcggagaatgccggacagagaggcatggctctggaggaattctgccaaatgggacagggcaagctgccgcctctccacaacctggctggcctcctcaaacagctggaagcagtcctcagcctttccctgcaggaggtggaggtcctcagcacggcccagagaacccaactttgctaagtgaccctgcagactctgcaattcgccctttttgctctctacttctgctgcgtggtccttatgccgagtaagggctacttgatggtccattatgctaatctcagaggtagtttgtaattcactgagaaacagtttaatccagacagaaaaggaaagcagcagctcatcaaattgctggtgttcagcaaccacagactgaagaaaattaatccttttgttaatgatctgtggtaaatctctccatctctcatccaactgctccaaatgtagtttcatcattttcacatcatctttggaggctactgagaacaatgattccttcaattgcaaaagtttgctatagaatgaggcctgggatacaacttcattttgcagtgcctgtattaactgaagttcaccttccactttgactctgtctgcagaaatgtccatttctggggaactggctttagcttcaccccgctctaaccaggtcaaaaaggatgatagttctttctctagcctctgccagtgggccagcagattctccagcgccgtctgtctctccttcgccctccttaggatgtcctcgtattgctgctgtagagccgcagcctcctgaacacaggaatctctgttcacaaccttcctggcactggctgagaaggcagtgatcgcgctgctcagtgactccagggcctggcagagatccatatgttcttgaagaactttgtatgtttctgtagctgaagaacatattttaattggaacagcaagtttatcttcaaattcagacacagattgctggatctttctaaggttctcttcaaacttttgctgctgagataaatgtcccaggattgttccttccagacactgtgcatgctctcgaagctcttccccgtatcttcttatttgtgtcaacttggctttaattcgagcagattctccagtggtaacaaactgagcaaaagactgggcttcttcttctaatcctacaatgctgctgagcttactttctatttcctgaattgtgaccttaatttggctgatttgcatgtccatggcagatgacgaagtttccaaggcattgagttctttttctttctcagttatccagacggacagagtctcaaaattactgccaaaatgatcccacttggttttcaccatttccatggttttaatatcttcttcaagcgtgtcttctaattttttgacttgttctttgattgacttggcctgctgttgaagcagctgcttattttggggcccaagcggtatctctgaagcttcctttacaaggttctcagcctggactgcaatactttctgtccgtttagaaaactcctttgtttgttccagttctgaagataaactttccaaactgctaaaactcaagaagcgttcatgactggaacctgtttgaaaaaggtatcttactactgtttctttgtttgtttcaaatcgctcccattttcttaatgtgacctggatgcggcgttcctgcctctcccggctgcgctccaggccatccagtgtgctctccagcttccgcagctcctcgtggcctcggtcaggcagccccccttctccctgctgcgcctgcgcgatctgctgctgcacatctctcttctttgctgagatccgctttgtcttttgctggtgatgaagaagtaactgctgtgcttcaaacagattttcagtatccaagatcttctcagcttgttcctggacttctttagagccagaaattaattcttcgagagaatttttgactatttctttgtactggacacagtccccaaaattgcttagcatcttttcaacctctgacagcagcgtcacaagagccttgaaagagctggataattttgccagctcatctccctgcttttgggcttcattctcagaagaaacttctgtcaaaactttcagcctggatttcagccagctgagggtctcaccccttttggtaacaccatttctgatctcttcaacggcacgtttaacctctccgtggttggcagtatcgatggcctcacccttgatcccctttaattgtgtctcatttgtagatatccaagatgagaactcagagaatctgctagtgtagtccttccacttgtctgggtcttccatgagcttcctgtaggtgctgtcaatggcagctctgagctctttgagagtcacgtgacaggttccaggtgtgtcccttactgggtcccgcactgggagtttcacacagagttcctcgatgagctgtaaccttttctcacagagatgatgaggacctttgtcactgaagaaaaccctgtgctctttaattatcttttcactgccttcctggggcatcagcttggtctctcgatccagctcagttctgcattcttctacagaggctaagaacctattcttctccacatcaatcttcagatgaagcaaatgataaggggcttctccttgaagatccttccattgtttgtggagctttcgaacagcttcctgcagcccctgctgctcctgctctggaaggatgtcggtgagttcatcacaagctttcaggaaagcattgagcaccctctgatccagctgactgaaaaactcagtgtgtctccgcaggagctcctctggatcccccttttcctccaggccctcctgagcaatccgcagtaccttctccaactctgctcgagactcctcaaacttcttcatcaagcgactgttggtttccacatgcttcttccaatctccagttttctttaccatactctgaaaagcaacatgaatatctgcaatctgtctttgtagcctcgtctgatcaaaatgctttaacacgttgctcaaggtcacaaacttttgaacactttgactgcctttctcaataagtgtcaaggttttcttacagttttcttgacaagctaacagttcctgatgtttttgtttaaaaagggcactcgattgtgcctcacgctcaagaactgtgataatttcattgattttcccaagtgagtcataaaaggacgtcatctgcttttctaattcctccaacggaatcaacagctgctgagactcataaaggagtggggagtaacattctttgaccttggttagctgctctttgagctttgacatggtcgcaaacatttcttttccttcttcttgggggctttctttggtaatgaggtgtgctgtctttgtaattatcttgtattgggcatccatcacaggcaccctctgctcaatatcctccaagtcttgaattaatagcttgacattcataaaagagacttctaagggttcagaaagtttcttatgggcttccgttgcaaaagcagacagggtaacaacacagtctgtgtattccttcttcattctgtccatctcatcagcttgagcatattgcttgacttccataaacaactccctccaccgcccatttagcaacagtaattgctgcttcaggtcacgggaaaccatctcatcacaggtttcaattagaaaattgccagcatcgttcatggcagtatgctgctgaatccaatgaggtaaatttcgaaaaaaatcctttttggcattttctgattgattgagcattttttcagcatcctctagccaggcttgcagactagccactgtattgccatagcgatcccagttagagatcacttcttccagcatgctcctcacactcctcacttctactgagagattcctccactgagcggtggtttcattcatgaatttcatcacattctcagcttcttccactgaaccatctgctttgacatacatctcagctgtctgtttcaagatctggtatgtcacctcatattgttcaaagaacttgctattttctataaaagacacgtagttttgtagaagctgctccactgactctctcctcccgtacttaatgatccaagacttcagctttgactctgcaagaaccagcagtgagagcagacggtactttaattctaaaaattccattttcattaggtgtagctctgatgtggaggaaacaaaatgaaacctctcggccatgtcctctaattgatcaggtggcactggaatcccgttaacagacctggtccggtagatttcatggaatgctcttttgtgggcatccgtgttttgaagcagatccttatgttgctcaagtttccgttgtatcgtgtttgctgtttcctcgtggacctgttgaacggttatttcctctctcagggccacctccgctctgtacagccaggcacctatggtgcccagaggtgcaggaagagatttatcaagctgtatatgccagtcaaagagcctggaggtcactctatcccaagattgttttaccaatgcttggtcaagtgacaatttaccgtctctgtgtaatggttgtattaaatgttcaatctgtttcctcttcatttcatattgaactctgaagtgcttaaatgactgatatttatcctgtaaatttgattccaccatctgtgctcttgtcaaatctctctcaaattgttctatccaaactttcatttccttaaaaattactctgtcttctctcttaaaattttgtacagaatttgcaaaagatgggaaacctggaagtatttcatcatcctcttgcccatcagtgcttgcattgtggatgtcaggataatgtttcagaaactgggctacataggtcataatagatttctcatctggtttatccacatcaacgtcttcaggatctagcagtcttgggatccccagttctgtttcggcgatagtgaaagcatcctccaaattttctcggttggatctgcctttcactgtctccaagtccaccaattccggtcgaatggcatgaataactgaatgaaaggcaaccccgcttctccaactcttcccaaaatcttttacttctattccagtctgcttgccagctgtgtactgaacccactttaataaagccttcttagcatttccttggatcttggtggtcaccttccgtttacttggtgggctgggagtctcagagctaactatgctgtccacggaggatgcgctgctggacaaagactggagctggggcaggttgctggtcaactcttcaatctggaaatatagaataatggtccacatcaatccaagaactattgagggtcggccatcagctatatcggtggagttaatgttgactaatttaatcggtgatcctctgtgcatggactttcttccttcgaggaacttgagtgccgtgccaatgttagccacagcatggattcgcttcatccggcgtccttgttcacaaggcagtttctgcccagacaggacctccagaagggcaagcagtttaacaccatctttcatgtcttcaaaaagatcgtccaccaccattggaggtttccgcttggccagatgagagttgatccattttgtgaaagttcgtttttgtactatctcttgctcatcttgcagcctctgcatcacattggcgatatcccgaggacaccgggaggcccctctggaggttgccatggtccctccggaagcacgaagccaacaccaagagactcttcactggaggcagcacagggctacaccactctagaaaacatgcttggacttttctagatctattctgtcataaatgaattccaggcctttgcagcactcaacaaggaggcagctctcccaaagactgaactgcttctttttcttcttccgttttaagactgtcctcttacatgaactcaagaaccttctctctcggcctcgttcagtttcccagcagcaaggcgaagcgagcgaacgcttcctcccggctctctgcgcccaggctcggcgggaccccggggatgcgcggctgtccgcccgccctgtcgccgggatcgggcgcggtctgcaggactgcgggagcccagccgccctcctggagatgcacggccttgggcgtttctccgcagctgcaaagctgtgctgtgacccacccgctcagcgagcctttataccgggaccacctcccgggggtcgaggtgggaaggaaatgtccctgagagccgggacgcgctgcctccgctgcctggaggagctgcgctgtcctgccagctaacttttgcccacggtttccactgcc

SEQ ID NO: 9572 - RNA, 14237 nt, Homo sapiens
  source 1..14237: mol_type = other RNA
agttcttcagtggcaagctttatcaaaatcttccttaaaatgcttcctagaaaccaaattcttctctagttcttgtaaccggtgactgcacttttgtaaaacactgtcatagacactctgcaattcctgaagcttccccagcacttcactcttttcctgctctgtgacttccttcattagttcgcgaccctgggcccaaagtccagtgacttcattttggtaagtcttgaggctggcttgtgcactcttacatgttttgacttgtttgctcacatcatctggtaacagacagatgtgttcacggaacattatctttcgctcatgttgctgaatttggctggtggcctggaacactgccatgagaaactgggttttctcggacaaggctttgtttaagtactttcttcgctggcccactaagtcactgagacaattcacgtggctttgtgcatcagagagagccttctggatgacctgtcgctcattgagaccaagatctgccatgaccctgtctgcgtcctttataagcgatttcaggagcatctgcttggcctccagttcactgcagatggccaggtgatccatgagaaggttctgagccatatctggaggagggctctgcttaagggcctcggcgatgttgggttgttgctcttctgcccactccattagctcctgaaatctggactgcaccacatttaactcctccaagttggtgactgacacttggattttccttttaatgaggtcctcaagctgaaaccaacgttgctctaaatgactcgtctgttctttgactaactccttgtcatctaaattcagatgctctatcattttctgcttttgatctttcagatcttcaatagcatactttctctcctgcaatgccaatgctaactttttcaaagcttccaggtggacagctgtactctctgcatcagatctggccaagttatcccattctgtagtaaatttttctaggaacacttcaacaacattcatacagtcatggtaatctcttgttctctgaagatcctcttccctttgcaagcacaggttgttagactgacggcacaaatcgagccactgatcatttaaatgatttatttccttgtgttcaggcgattcctccttctttgttaacttattcaccttttctattatggtgttcacggatgcctgtttgctctgtagtttcttaacaaaatccttaacttgtgaaaccatgttctgtgcaatgttcagctccagctcagagtgcctcctcttcatgttctgcagttgctgatcagcatcttgcaggtaaatccagagctcagacttcaggtgcttgatctcttcccagccctgagttaagttctgggcctggacaagcttttgttcaatcgtttgctctgtttgttgaatgtcttttgctgtggttttcaccgaagcatttgacaggtcacacatggagcaaaggagatctaggtaggtccttgcctgctcttgcaaagctctgaagtgtttgacctgcttaatggcttctgccctactaagaggtggttgaggacttggctctaaatccggctggactgcagaaagccaggcctggcactgctgcagggtgtcttgtcggctgacgtgcttctgaagttcgtgttccaaactctggtacatcctctgagctgtgctgcagatcgctgagtagctgtcctttgtgccctgcagatgagcatgcacgttttgtttaagtttcgcttgcaggtggtctgcacattggccaatcaaagtatcacctttcatttgaagattgttcaaacggtcttcaaaaccagcaatttcttccatcattgccttgtggtgggccaattgctgggtgattgtctccaggctgcttgtctccaggaggtcaggtgccaccagtctgccagacatctgcagcagccacttttcgacctcttggagctcactgttgtagtcttcatggtctttgactttcgcctccagactgaagacatgctcctttcctatgctgcacaggtcctggtaatcactttgaagttgatctattttgtcctttaaagtgacgtcctgcaccagttccaaaagagcttcacccttctctctcactgactttactgatggttcatgggacagcaccgtttgttgaagtgacttgtatttagataactgagcttttttctcatataattccattttgggttcttcaggaacatgtagaatttcctggtattctgctatccactgtgtcagtgctttgcatttatctgagaattcctttgctaaatgaagacctttttccagcgtcatgtgttctttccggacagtgctggtcagttccttcaactgctccatgtgatcatgaatctcctttcttaacctctctgcctcgccttcctccaagtatttaacagccctctctcctttctcccgggctgatttcagcaaactgtgacctttctccatgtctttgagcaaaacctccaacgtcttcaatttcttccccatcattactgtatctactttgtcaatcttggtagccacattcttgaagtttttatgagtagagccataccaatcagaataggaactgagggatgattctgattcctccaaactctgaatctcctcctccaggaattttatttgttccagcacttggagaagcagggcctggtatctggaagtcagctgggtggcctggcaacccattctgctgttcacgtggctctcgtccagtatctcctgagctctagctcccacttcctcaacttcatctctgtatgcagtcacttcttcgtgccacttcttcatctgatgtaattgtatctccttggttgccctgttagactgacgtctggtcctgggactaactttctcctctgctgttttgagccattcatctacttgctgaaacttttgctccattagcctcaatttgttcaccacgttattgaactgagttcgagtctcggacagcctgtgctggtaagcctgccagtcttgccggagagactctaaagcccggtcctctgcctgtgggatacctgatgggatcacatcctctctggtgtgcagcactgagttcaacagggcctgcccctctgcacagtgtacctgtagctcctgaagatcacgcaatgttgtctcatgagtgtgggcatcaccttcaagaactgaatactggtcgagcttttcttgttcttgccccaaccaaacttcaaatgcctttaggtctctctgatactcttggtgcaggcggacaagtttttcagacttggttacggcttccttggccctctcttggatggctctgtatcgttcctgtagatcctggagttctagctgggtgacatagtgttctgtcatgccagcccctttgacttcgatggtctccagcaagctgctgtaactcagcacttcttcatttaataacttggcttttccgagcatcgttgttttatcccgcagctccgcatgctgcctttctgattcattcaggttggcttccatactatccatccaaccggagaactgtcgaacgccatcctgataacttgtccacttggagagagctccttcgagttggcttttacaacgaatccctgcagacaaaagggatgcccacatatccttcacactctgcagctgctgctgaatagtgggaatgccttctggagaagtattctgaaggacagattctcccctggtcactatcattttcatctgaatctctttttcctgtttgactgataatagagcctcgagcttgagcgtcctgctgtccagcacacttttgtcggatgtcgggtggcagtatgaatccagcatgtgaatcgcatccgtcatccagtcttgtaattctttaatcccaagagagaactgattgtgttctgcaacgattctatccagtcttgacactttctcctttgttaaattgcttagcgctagatactgagaagacagctgcgacactctgtgcctaaagctcttgctggcagcttgtccttcccacagctgctgagctttctctttcagcctgttgagctgaggctcgtagcagtgtatttcctcaaggacagactggagcttctgctgctccctcctctttgctggcagatcatagaggcgattgctgctttcatggaccatcttctcagttttactcagccagtcctggataggctcagcacttacttcaaagtccttcatttggatctttagattctctagagcagattctttttggtggagatttgaatgaaaatttttccaatcttcttttgcagctgtaactttggcctggatccctttcgctttctctttggtcagcagggtactcagaagttcccctttagacagcatcatgtttagcttgtgctgtccattttcactttctgacaaaaactcctgtattttctgaagactagttgaaacttcacttatattttgaggtatatcaaaacacttggcggtagtgatttttgcattaaccaaccactgctggaaatccctgaaggcctttcgaaatctttgctgtaaaatctgttctttattctggcagcccttggatgcttgcaaacaaagacaattatactctttaatcaagccagaaacttttccactgtaggtactcaggtctctggaaaatcgacaaagttcattcagctgagacttgagatcctctgttctaggctctgctttttgcaaagcatccagtatctcttgtcctttgtgccagcattccactatctcctcatccgtgttcttgccttccaggagggttaactgctgagcccaggttttcagaagggcactgaactgttccagggcctgctccagttgagccacttggcctgagaattcctgctccgaaagggccatctggctgaccaggttctccaaacagctctgcgtttggaatacactgtcttcccactgcttccagtcggcacgcagggcctgcatctccgtgtgcatgagctcacacccactggcagttgtgttctgtttcacttcgggagccagcgactccactctgctgagacggcttgcaccaatctctctggaatctatcagctccttaatttttgataactttttctgggtggctgatgaatctccagacatatctgaccaccggtgaagttcttcctttgctgaatggagccaatctgtgaactcgtggaccgcatctaaatacattagatgatctttcacaatctcttccactttcctcattttttccttggcaacagtcattatatcattaaactgtgttttcagctcctcttgagctgtgtccttgaaagactcatcctctgtcttttcgtagagctccctggacttcgcaattagacggtgaagggctctcgtgtgatcttctgcctcagacaggatggactggaggtggtcaagcaggacgaacttctctttcagacctggctgtggttgtaagggatgttctattttttgatccactgattccatccactgctccaactggtttttcctctctacatagtcattccattggctaatcacagactctaaagtgctttgagcgtggacggaggagctcatgatgtcagcccacacttctttaagggtctctaactgagtctgaatcaccctctgaccttctttgttgctacttctcaaggcctgttcccccttgccaatggccatattcaacttaacttccccttcacctttcatcaggagaatatcctgtatttgtgacagccgtttctccagggtgtctttgctcccaagagtgctctctgcacaggccagtctgtcctgaatggccttcacccagaaccacatgctttgcagtgcttcctccagggcttcgtgctcctgaagggccacctggcagctccggagtttctctttggtcattctaagtaggttctggtggcttgtgaggagctgggaacacaggcggccctcctgcccagcaccgtggccttcttcactcagaagctgccctctctgggaaagcttatcaagagactctcttgcagccagcagttctcccaaaaacatttcaactttatgaacttcatttttcttctcaggaatgtgctgtttactctctcccaagttttccgtattgaacctttcttccatttcatggatccataagttcagttttctgtgctgatcttcaaagcttccaagttctgaagcacagtcttgaagagcctgcttatctttaaggcattgtttcagaaatgcttgaaactcttcattggcctttgtgatttgttcttgaatgctactgacaatttgtttagacaaatgtgcatacaaagtttgtccttcttgagtcactgcatcaagtttgctctgcccatcactgactgagtccaaaatgttctgaagatcatggagctttgcttctagaactttgctgtcaccggtgcgatctgatgattcttttgctgctgcctttgctcccaaaaaccattcttggaattcctgcatagactcactgaagtgtttttccagagattcctgcaggctggcctgggttttggagcacaactggctcacggcttcatgtttctttatcagaccagtcattgcacggcccaggctctccaactcagctgagtggtacttgcggcacaagctattgagattttcttgggtagagctgatgttgctttgttgactttgaagttctttttgtatatccttgacttttttcaatgcttcacaagtctcattttgggcacagttcatcaacgattcttccacttttgtgaaccatgttgttatgtcattaataaacttctccacttgtgtactttgagccgtgaaatccttcagggttccttttgctacttcagttatttctttggcatgctccagtttctgcattaagtctgcttctataaactgaaggtctggcggtgtttctagatttttagttaattctttcagatcattaactttggaatgcagttcttccaatctcaatgctttgtttttaacttcagactcaaattctttaagcagttcttcagctctgaggtggttatccaggttgctgatgttttctgccatctgtggaacgcagttgtttgaccatccctcaatctcatctctagttgacagtacatcatcccaaatggacaggcttactctcagcctatccatgttttcttcaagtttctctgatacatccagccatttgtccacggtgctctccatgtctgttttcaccaagctgaaatcactactgtgaattttcttcagctcagataacaagtgttttcctttgctggtaaagttatccaagtctttctgtttgtaattcattttgttcttggcagtttcatgcttggaaaaagcccatttaagatcctcctgatcttttatggtagttctggttacaatcacactgctggcattttctaagactttagatacagctgatttcaggttctgatattctctcattaagtcaataagtccacagcactgaccctgattttcatgaattagtcttttggtatcatcccaggtgacctctaagcggtttatctccctgtcaacttcaggtgcaaaagctacatctttctgggcaatttgcttggctttgtctttcaaccaacatagttcatgctcgtgagaattcaattcatcttctagctgattaaacactcttaacctctgctgaagagcttggcgggtaggttctttcaatcgctctttgtcagtcctttcttcaatgtcctcaatgcttttcagaagctcctctttctggtcttggaatgcttttttcaacactgccagagcatctgcctcactctgcttggttcccagaaggttctggatcctctctacctctccacagagctgatcagccgtggctctgcaggaagtcctttgctcagagctcccgattttcagatggtattgggctttggaaagaatgccatccagactgacggcagcagattctaatgctttagcattttgaagagcatcattgaggtccttttctatcaaatcagactcgttcttattcatactgttggttgcttccactgtttgcctcagctggcggagaatgccggacagagaggcatggctctggaggaattctgccaaatgggacagggcaagctgccgcctctccacaacctggctggcctcctcaaacagctggaagcagtcctcagcctttccctgcaggaggtggaggtcctcagcacggcccagagaacccaactttgctaagtgaccctgcagactctgcaattcgccctttttgctctctacttctgctgcgtggtccttatgccgagtaagggctacttgatggtccattatgctaatctcagaggtagtttgtaattcactgagaaacagtttaatccagacagaaaaggaaagcagcagctcatcaaattgctggtgttcagcaaccacagactgaagaaaattaatccttttgttaatgatctgtggtaaatctctccatctctcatccaactgctccaaatgtagtttcatcattttcacatcatctttggaggctactgagaacaatgattccttcaattgcaaaagtttgctatagaatgaggcctgggatacaacttcattttgcagtgcctgtattaactgaagttcaccttccactttgactctgtctgcagaaatgtccatttctggggaactggctttagcttcaccccgctctaaccaggtcaaaaaggatgatagttctttctctagcctctgccagtgggccagcagattctccagcgccgtctgtctctccttcgccctccttaggatgtcctcgtattgctgctgtagagccgcagcctcctgaacacaggaatctctgttcacaaccttcctggcactggctgagaaggcagtgatcgcgctgctcagtgactccagggcctggcagagatccatatgttcttgaagaactttgtatgtttctgtagctgaagaacatattttaattggaacagcaagtttatcttcaaattcagacacagattgctggatctttctaaggttctcttcaaacttttgctgctgagataaatgtcccaggattgttccttccagacactgtgcatgctctcgaagctcttccccgtatcttcttatttgtgtcaacttggctttaattcgagcagattctccagtggtaacaaactgagcaaaagactgggcttcttcttctaatcctacaatgctgctgagcttactttctatttcctgaattgtgaccttaatttggctgatttgcatgtccatggcagatgacgaagtttccaaggcattgagttctttttctttctcagttatccagacggacagagtctcaaaattactgccaaaatgatcccacttggttttcaccatttccatggttttaatatcttcttcaagcgtgtcttctaattttttgacttgttctttgattgacttggcctgctgttgaagcagctgcttattttggggcccaagcggtatctctgaagcttcctttacaaggttctcagcctggactgcaatactttctgtccgtttagaaaactcctttgtttgttccagttctgaagataaactttccaaactgctaaaactcaagaagcgttcatgactggaacctgtttgaaaaaggtatcttactactgtttctttgtttgtttcaaatcgctcccattttcttaatgtgacctggatgcggcgttcctgcctctcccggctgcgctccaggccatccagtgtgctctccagcttccgcagctcctcgtggcctcggtcaggcagccccccttctccctgctgcgcctgcgcgatctgctgctgcacatctctcttctttgctgagatccgctttgtcttttgctggtgatgaagaagtaactgctgtgcttcaaacagattttcagtatccaagatcttctcagcttgttcctggacttctttagagccagaaattaattcttcgagagaatttttgactatttctttgtactggacacagtccccaaaattgcttagcatcttttcaacctctgacagcagcgtcacaagagccttgaaagagctggataattttgccagctcatctccctgcttttgggcttcattctcagaagaaacttctgtcaaaactttcagcctggatttcagccagctgagggtctcaccccttttggtaacaccatttctgatctcttcaacggcacgtttaacctctccgtggttggcagtatcgatggcctcacccttgatcccctttaattgtgtctcatttgtagatatccaagatgagaactcagagaatctgctagtgtagtccttccacttgtctgggtcttccatgagcttcctgtaggtgctgtcaatggcagctctgagctctttgagagtcacgtgacaggttccaggtgtgtcccttactgggtcccgcactgggagtttcacacagagttcctcgatgagctgtaaccttttctcacagagatgatgaggacctttgtcactgaagaaaaccctgtgctctttaattatcttttcactgccttcctggggcatcagcttggtctctcgatccagctcagttctgcattcttctacagaggctaagaacctattcttctccacatcaatcttcagatgaagcaaatgataaggggcttctccttgaagatccttccattgtttgtggagctttcgaacagcttcctgcagcccctgctgctcctgctctggaaggatgtcggtgagttcatcacaagctttcaggaaagcattgagcaccctctgatccagctgactgaaaaactcagtgtgtctccgcaggagctcctctggatcccccttttcctccaggccctcctgagcaatccgcagtaccttctccaactctgctcgagactcctcaaacttcttcatcaagcgactgttggtttccacatgcttcttccaatctccagttttctttaccatactctgaaaagcaacatgaatatctgcaatctgtctttgtagcctcgtctgatcaaaatgctttaacacgttgctcaaggtcacaaacttttgaacactttgactgcctttctcaataagtgtcaaggttttcttacagttttcttgacaagctaacagttcctgatgtttttgtttaaaaagggcactcgattgtgcctcacgctcaagaactgtgataatttcattgattttcccaagtgagtcataaaaggacgtcatctgcttttctaattcctccaacggaatcaacagctgctgagactcataaaggagtggggagtaacattctttgaccttggttagctgctctttgagctttgacatggtcgcaaacatttcttttccttcttcttgggggctttctttggtaatgaggtgtgctgtctttgtaattatcttgtattgggcatccatcacaggcaccctctgctcaatatcctccaagtcttgaattaatagcttgacattcataaaagagacttctaagggttcagaaagtttcttatgggcttccgttgcaaaagcagacagggtaacaacacagtctgtgtattccttcttcattctgtccatctcatcagcttgagcatattgcttgacttccataaacaactccctccaccgcccatttagcaacagtaattgctgcttcaggtcacgggaaaccatctcatcacaggtttcaattagaaaattgccagcatcgttcatggcagtatgctgctgaatccaatgaggtaaatttcgaaaaaaatcctttttggcattttctgattgattgagcattttttcagcatcctctagccaggcttgcagactagccactgtattgccatagcgatcccagttagagatcacttcttccagcatgctcctcacactcctcacttctactgagagattcctccactgagcggtggtttcattcatgaatttcatcacattctcagcttcttccactgaaccatctgctttgacatacatctcagctgtctgtttcaagatctggtatgtcacctcatattgttcaaagaacttgctattttctataaaagacacgtagttttgtagaagctgctccactgactctctcctcccgtacttaatgatccaagacttcagctttgactctgcaagaaccagcagtgagagcagacggtactttaattctaaaaattccattttcattaggtgtagctctgatgtggaggaaacaaaatgaaacctctcggccatgtcctctaattgatcaggtggcactggaatcccgttaacagacctggtccggtagatttcatggaatgctcttttgtgggcatccgtgttttgaagcagatccttatgttgctcaagtttccgttgtatcgtgtttgctgtttcctcgtggacctgttgaacggttatttcctctctcagggccacctccgctctgtacagccaggcacctatggtgcccagaggtgcaggaagagatttatcaagctgtatatgccagtcaaagagcctggaggtcactctatcccaagattgttttaccaatgcttggtcaagtgacaatttaccgtctctgtgtaatggttgtattaaatgttcaatctgtttcctcttcatttcatattgaactctgaagtgcttaaatgactgatatttatcctgtaaatttgattccaccatctgtgctcttgtcaaatctctctcaaattgttctatccaaactttcatttccttaaaaattactctgtcttctctcttaaaattttgtacagaatttgcaaaagatgggaaacctggaagtatttcatcatcctcttgcccatcagtgcttgcattgtggatgtcaggataatgtttcagaaactgggctacataggtcataatagatttctcatctggtttatccacatcaacgtcttcaggatctagcagtcttgggatccccagttctgtttcggcgatagtgaaagcatcctccaaattttctcggttggatctgcctttcactgtctccaagtccaccaattccggtcgaatggcatgaataactgaatgaaaggcaaccccgcttctccaactcttcccaaaatcttttacttctattccagtctgcttgccagctgtgtactgaacccactttaataaagccttcttagcatttccttggatcttggtggtcaccttccgtttacttggtgggctgggagtctcagagctaactatgctgtccacggaggatgcgctgctggacaaagactggagctggggcaggttgctggtcaactcttcaatctggaaatatagaataatggtccacatcaatccaagaactattgagggtcggccatcagctatatcggtggagttaatgttgactaatttaatcggtgatcctctgtgcatggactttcttccttcgaggaacttgagtgccgtgccaatgttagccacagcatggattcgcttcatccggcgtccttgttcacaaggcagtttctgcccagacaggacctccagaagggcaagcagtttaacaccatctttcatgtcttcaaaaagatcgtccaccaccattggaggtttccgcttggccagatgagagttgatccattttgtgaaagttcgtttttgtactatctcttgctcatcttgcagcctctgcatcacattggcgatatcccgaggacaccgggaggcccctctggaggttgccatggtccctccggaagcacgaagccaacaccaagagactcttcactggaggcagcacagggctacaccactctagaaaacatgcttggacttttctagatctattctgtcataaatgaattccaggcctttgcagcactcaacaaggaggcagctctcccaaagactgaactgcttctttttcttcttccgttttaagactgtcctcttacatgaactcaagaaccttctctctcggcctcgttcagtttcccagcagcaaggcgaagcgagcgaacgcttcctcccggctctctgcgcccaggctcggcgggaccccggggatgcgcggctgtccgcccgccctgtcgccgggatcgggcgcggtctgcaggactgcgggagcccagccgccctggtgacagaggacaacaatctcagcccgctgcggccggcggccgcggcccggcgcccgcgctcaccctggctggctcgcccacact

SEQ ID NO: 9573 - RNA, 14241 nt, Homo sapiens
  source 1..14241: mol_type = other RNA
agttcttcagtggcaagctttatcaaaatcttccttaaaatgcttcctagaaaccaaattcttctctagttcttgtaaccggtgactgcacttttgtaaaacactgtcatagacactctgcaattcctgaagcttccccagcacttcactcttttcctgctctgtgacttccttcattagttcgcgaccctgggcccaaagtccagtgacttcattttggtaagtcttgaggctggcttgtgcactcttacatgttttgacttgtttgctcacatcatctggtaacagacagatgtgttcacggaacattatctttcgctcatgttgctgaatttggctggtggcctggaacactgccatgagaaactgggttttctcggacaaggctttgtttaagtactttcttcgctggcccactaagtcactgagacaattcacgtggctttgtgcatcagagagagccttctggatgacctgtcgctcattgagaccaagatctgccatgaccctgtctgcgtcctttataagcgatttcaggagcatctgcttggcctccagttcactgcagatggccaggtgatccatgagaaggttctgagccatatctggaggagggctctgcttaagggcctcggcgatgttgggttgttgctcttctgcccactccattagctcctgaaatctggactgcaccacatttaactcctccaagttggtgactgacacttggattttccttttaatgaggtcctcaagctgaaaccaacgttgctctaaatgactcgtctgttctttgactaactccttgtcatctaaattcagatgctctatcattttctgcttttgatctttcagatcttcaatagcatactttctctcctgcaatgccaatgctaactttttcaaagcttccaggtggacagctgtactctctgcatcagatctggccaagttatcccattctgtagtaaatttttctaggaacacttcaacaacattcatacagtcatggtaatctcttgttctctgaagatcctcttccctttgcaagcacaggttgttagactgacggcacaaatcgagccactgatcatttaaatgatttatttccttgtgttcaggcgattcctccttctttgttaacttattcaccttttctattatggtgttcacggatgcctgtttgctctgtagtttcttaacaaaatccttaacttgtgaaaccatgttctgtgcaatgttcagctccagctcagagtgcctcctcttcatgttctgcagttgctgatcagcatcttgcaggtaaatccagagctcagacttcaggtgcttgatctcttcccagccctgagttaagttctgggcctggacaagcttttgttcaatcgtttgctctgtttgttgaatgtcttttgctgtggttttcaccgaagcatttgacaggtcacacatggagcaaaggagatctaggtaggtccttgcctgctcttgcaaagctctgaagtgtttgacctgcttaatggcttctgccctactaagaggtggttgaggacttggctctaaatccggctggactgcagaaagccaggcctggcactgctgcagggtgtcttgtcggctgacgtgcttctgaagttcgtgttccaaactctggtacatcctctgagctgtgctgcagatcgctgagtagctgtcctttgtgccctgcagatgagcatgcacgttttgtttaagtttcgcttgcaggtggtctgcacattggccaatcaaagtatcacctttcatttgaagattgttcaaacggtcttcaaaaccagcaatttcttccatcattgccttgtggtgggccaattgctgggtgattgtctccaggctgcttgtctccaggaggtcaggtgccaccagtctgccagacatctgcagcagccacttttcgacctcttggagctcactgttgtagtcttcatggtctttgactttcgcctccagactgaagacatgctcctttcctatgctgcacaggtcctggtaatcactttgaagttgatctattttgtcctttaaagtgacgtcctgcaccagttccaaaagagcttcacccttctctctcactgactttactgatggttcatgggacagcaccgtttgttgaagtgacttgtatttagataactgagcttttttctcatataattccattttgggttcttcaggaacatgtagaatttcctggtattctgctatccactgtgtcagtgctttgcatttatctgagaattcctttgctaaatgaagacctttttccagcgtcatgtgttctttccggacagtgctggtcagttccttcaactgctccatgtgatcatgaatctcctttcttaacctctctgcctcgccttcctccaagtatttaacagccctctctcctttctcccgggctgatttcagcaaactgtgacctttctccatgtctttgagcaaaacctccaacgtcttcaatttcttccccatcattactgtatctactttgtcaatcttggtagccacattcttgaagtttttatgagtagagccataccaatcagaataggaactgagggatgattctgattcctccaaactctgaatctcctcctccaggaattttatttgttccagcacttggagaagcagggcctggtatctggaagtcagctgggtggcctggcaacccattctgctgttcacgtggctctcgtccagtatctcctgagctctagctcccacttcctcaacttcatctctgtatgcagtcacttcttcgtgccacttcttcatctgatgtaattgtatctccttggttgccctgttagactgacgtctggtcctgggactaactttctcctctgctgttttgagccattcatctacttgctgaaacttttgctccattagcctcaatttgttcaccacgttattgaactgagttcgagtctcggacagcctgtgctggtaagcctgccagtcttgccggagagactctaaagcccggtcctctgcctgtgggatacctgatgggatcacatcctctctggtgtgcagcactgagttcaacagggcctgcccctctgcacagtgtacctgtagctcctgaagatcacgcaatgttgtctcatgagtgtgggcatcaccttcaagaactgaatactggtcgagcttttcttgttcttgccccaaccaaacttcaaatgcctttaggtctctctgatactcttggtgcaggcggacaagtttttcagacttggttacggcttccttggccctctcttggatggctctgtatcgttcctgtagatcctggagttctagctgggtgacatagtgttctgtcatgccagcccctttgacttcgatggtctccagcaagctgctgtaactcagcacttcttcatttaataacttggcttttccgagcatcgttgttttatcccgcagctccgcatgctgcctttctgattcattcaggttggcttccatactatccatccaaccggagaactgtcgaacgccatcctgataacttgtccacttggagagagctccttcgagttggcttttacaacgaatccctgcagacaaaagggatgcccacatatccttcacactctgcagctgctgctgaatagtgggaatgccttctggagaagtattctgaaggacagattctcccctggtcactatcattttcatctgaatctctttttcctgtttgactgataatagagcctcgagcttgagcgtcctgctgtccagcacacttttgtcggatgtcgggtggcagtatgaatccagcatgtgaatcgcatccgtcatccagtcttgtaattctttaatcccaagagagaactgattgtgttctgcaacgattctatccagtcttgacactttctcctttgttaaattgcttagcgctagatactgagaagacagctgcgacactctgtgcctaaagctcttgctggcagcttgtccttcccacagctgctgagctttctctttcagcctgttgagctgaggctcgtagcagtgtatttcctcaaggacagactggagcttctgctgctccctcctctttgctggcagatcatagaggcgattgctgctttcatggaccatcttctcagttttactcagccagtcctggataggctcagcacttacttcaaagtccttcatttggatctttagattctctagagcagattctttttggtggagatttgaatgaaaatttttccaatcttcttttgcagctgtaactttggcctggatccctttcgctttctctttggtcagcagggtactcagaagttcccctttagacagcatcatgtttagcttgtgctgtccattttcactttctgacaaaaactcctgtattttctgaagactagttgaaacttcacttatattttgaggtatatcaaaacacttggcggtagtgatttttgcattaaccaaccactgctggaaatccctgaaggcctttcgaaatctttgctgtaaaatctgttctttattctggcagcccttggatgcttgcaaacaaagacaattatactctttaatcaagccagaaacttttccactgtaggtactcaggtctctggaaaatcgacaaagttcattcagctgagacttgagatcctctgttctaggctctgctttttgcaaagcatccagtatctcttgtcctttgtgccagcattccactatctcctcatccgtgttcttgccttccaggagggttaactgctgagcccaggttttcagaagggcactgaactgttccagggcctgctccagttgagccacttggcctgagaattcctgctccgaaagggccatctggctgaccaggttctccaaacagctctgcgtttggaatacactgtcttcccactgcttccagtcggcacgcagggcctgcatctccgtgtgcatgagctcacacccactggcagttgtgttctgtttcacttcgggagccagcgactccactctgctgagacggcttgcaccaatctctctggaatctatcagctccttaatttttgataactttttctgggtggctgatgaatctccagacatatctgaccaccggtgaagttcttcctttgctgaatggagccaatctgtgaactcgtggaccgcatctaaatacattagatgatctttcacaatctcttccactttcctcattttttccttggcaacagtcattatatcattaaactgtgttttcagctcctcttgagctgtgtccttgaaagactcatcctctgtcttttcgtagagctccctggacttcgcaattagacggtgaagggctctcgtgtgatcttctgcctcagacaggatggactggaggtggtcaagcaggacgaacttctctttcagacctggctgtggttgtaagggatgttctattttttgatccactgattccatccactgctccaactggtttttcctctctacatagtcattccattggctaatcacagactctaaagtgctttgagcgtggacggaggagctcatgatgtcagcccacacttctttaagggtctctaactgagtctgaatcaccctctgaccttctttgttgctacttctcaaggcctgttcccccttgccaatggccatattcaacttaacttccccttcacctttcatcaggagaatatcctgtatttgtgacagccgtttctccagggtgtctttgctcccaagagtgctctctgcacaggccagtctgtcctgaatggccttcacccagaaccacatgctttgcagtgcttcctccagggcttcgtgctcctgaagggccacctggcagctccggagtttctctttggtcattctaagtaggttctggtggcttgtgaggagctgggaacacaggcggccctcctgcccagcaccgtggccttcttcactcagaagctgccctctctgggaaagcttatcaagagactctcttgcagccagcagttctcccaaaaacatttcaactttatgaacttcatttttcttctcaggaatgtgctgtttactctctcccaagttttccgtattgaacctttcttccatttcatggatccataagttcagttttctgtgctgatcttcaaagcttccaagttctgaagcacagtcttgaagagcctgcttatctttaaggcattgtttcagaaatgcttgaaactcttcattggcctttgtgatttgttcttgaatgctactgacaatttgtttagacaaatgtgcatacaaagtttgtccttcttgagtcactgcatcaagtttgctctgcccatcactgactgagtccaaaatgttctgaagatcatggagctttgcttctagaactttgctgtcaccggtgcgatctgatgattcttttgctgctgcctttgctcccaaaaaccattcttggaattcctgcatagactcactgaagtgtttttccagagattcctgcaggctggcctgggttttggagcacaactggctcacggcttcatgtttctttatcagaccagtcattgcacggcccaggctctccaactcagctgagtggtacttgcggcacaagctattgagattttcttgggtagagctgatgttgctttgttgactttgaagttctttttgtatatccttgacttttttcaatgcttcacaagtctcattttgggcacagttcatcaacgattcttccacttttgtgaaccatgttgttatgtcattaataaacttctccacttgtgtactttgagccgtgaaatccttcagggttccttttgctacttcagttatttctttggcatgctccagtttctgcattaagtctgcttctataaactgaaggtctggcggtgtttctagatttttagttaattctttcagatcattaactttggaatgcagttcttccaatctcaatgctttgtttttaacttcagactcaaattctttaagcagttcttcagctctgaggtggttatccaggttgctgatgttttctgccatctgtggaacgcagttgtttgaccatccctcaatctcatctctagttgacagtacatcatcccaaatggacaggcttactctcagcctatccatgttttcttcaagtttctctgatacatccagccatttgtccacggtgctctccatgtctgttttcaccaagctgaaatcactactgtgaattttcttcagctcagataacaagtgttttcctttgctggtaaagttatccaagtctttctgtttgtaattcattttgttcttggcagtttcatgcttggaaaaagcccatttaagatcctcctgatcttttatggtagttctggttacaatcacactgctggcattttctaagactttagatacagctgatttcaggttctgatattctctcattaagtcaataagtccacagcactgaccctgattttcatgaattagtcttttggtatcatcccaggtgacctctaagcggtttatctccctgtcaacttcaggtgcaaaagctacatctttctgggcaatttgcttggctttgtctttcaaccaacatagttcatgctcgtgagaattcaattcatcttctagctgattaaacactcttaacctctgctgaagagcttggcgggtaggttctttcaatcgctctttgtcagtcctttcttcaatgtcctcaatgcttttcagaagctcctctttctggtcttggaatgcttttttcaacactgccagagcatctgcctcactctgcttggttcccagaaggttctggatcctctctacctctccacagagctgatcagccgtggctctgcaggaagtcctttgctcagagctcccgattttcagatggtattgggctttggaaagaatgccatccagactgacggcagcagattctaatgctttagcattttgaagagcatcattgaggtccttttctatcaaatcagactcgttcttattcatactgttggttgcttccactgtttgcctcagctggcggagaatgccggacagagaggcatggctctggaggaattctgccaaatgggacagggcaagctgccgcctctccacaacctggctggcctcctcaaacagctggaagcagtcctcagcctttccctgcaggaggtggaggtcctcagcacggcccagagaacccaactttgctaagtgaccctgcagactctgcaattcgccctttttgctctctacttctgctgcgtggtccttatgccgagtaagggctacttgatggtccattatgctaatctcagaggtagtttgtaattcactgagaaacagtttaatccagacagaaaaggaaagcagcagctcatcaaattgctggtgttcagcaaccacagactgaagaaaattaatccttttgttaatgatctgtggtaaatctctccatctctcatccaactgctccaaatgtagtttcatcattttcacatcatctttggaggctactgagaacaatgattccttcaattgcaaaagtttgctatagaatgaggcctgggatacaacttcattttgcagtgcctgtattaactgaagttcaccttccactttgactctgtctgcagaaatgtccatttctggggaactggctttagcttcaccccgctctaaccaggtcaaaaaggatgatagttctttctctagcctctgccagtgggccagcagattctccagcgccgtctgtctctccttcgccctccttaggatgtcctcgtattgctgctgtagagccgcagcctcctgaacacaggaatctctgttcacaaccttcctggcactggctgagaaggcagtgatcgcgctgctcagtgactccagggcctggcagagatccatatgttcttgaagaactttgtatgtttctgtagctgaagaacatattttaattggaacagcaagtttatcttcaaattcagacacagattgctggatctttctaaggttctcttcaaacttttgctgctgagataaatgtcccaggattgttccttccagacactgtgcatgctctcgaagctcttccccgtatcttcttatttgtgtcaacttggctttaattcgagcagattctccagtggtaacaaactgagcaaaagactgggcttcttcttctaatcctacaatgctgctgagcttactttctatttcctgaattgtgaccttaatttggctgatttgcatgtccatggcagatgacgaagtttccaaggcattgagttctttttctttctcagttatccagacggacagagtctcaaaattactgccaaaatgatcccacttggttttcaccatttccatggttttaatatcttcttcaagcgtgtcttctaattttttgacttgttctttgattgacttggcctgctgttgaagcagctgcttattttggggcccaagcggtatctctgaagcttcctttacaaggttctcagcctggactgcaatactttctgtccgtttagaaaactcctttgtttgttccagttctgaagataaactttccaaactgctaaaactcaagaagcgttcatgactggaacctgtttgaaaaaggtatcttactactgtttctttgtttgtttcaaatcgctcccattttcttaatgtgacctggatgcggcgttcctgcctctcccggctgcgctccaggccatccagtgtgctctccagcttccgcagctcctcgtggcctcggtcaggcagccccccttctccctgctgcgcctgcgcgatctgctgctgcacatctctcttctttgctgagatccgctttgtcttttgctggtgatgaagaagtaactgctgtgcttcaaacagattttcagtatccaagatcttctcagcttgttcctggacttctttagagccagaaattaattcttcgagagaatttttgactatttctttgtactggacacagtccccaaaattgcttagcatcttttcaacctctgacagcagcgtcacaagagccttgaaagagctggataattttgccagctcatctccctgcttttgggcttcattctcagaagaaacttctgtcaaaactttcagcctggatttcagccagctgagggtctcaccccttttggtaacaccatttctgatctcttcaacggcacgtttaacctctccgtggttggcagtatcgatggcctcacccttgatcccctttaattgtgtctcatttgtagatatccaagatgagaactcagagaatctgctagtgtagtccttccacttgtctgggtcttccatgagcttcctgtaggtgctgtcaatggcagctctgagctctttgagagtcacgtgacaggttccaggtgtgtcccttactgggtcccgcactgggagtttcacacagagttcctcgatgagctgtaaccttttctcacagagatgatgaggacctttgtcactgaagaaaaccctgtgctctttaattatcttttcactgccttcctggggcatcagcttggtctctcgatccagctcagttctgcattcttctacagaggctaagaacctattcttctccacatcaatcttcagatgaagcaaatgataaggggcttctccttgaagatccttccattgtttgtggagctttcgaacagcttcctgcagcccctgctgctcctgctctggaaggatgtcggtgagttcatcacaagctttcaggaaagcattgagcaccctctgatccagctgactgaaaaactcagtgtgtctccgcaggagctcctctggatcccccttttcctccaggccctcctgagcaatccgcagtaccttctccaactctgctcgagactcctcaaacttcttcatcaagcgactgttggtttccacatgcttcttccaatctccagttttctttaccatactctgaaaagcaacatgaatatctgcaatctgtctttgtagcctcgtctgatcaaaatgctttaacacgttgctcaaggtcacaaacttttgaacactttgactgcctttctcaataagtgtcaaggttttcttacagttttcttgacaagctaacagttcctgatgtttttgtttaaaaagggcactcgattgtgcctcacgctcaagaactgtgataatttcattgattttcccaagtgagtcataaaaggacgtcatctgcttttctaattcctccaacggaatcaacagctgctgagactcataaaggagtggggagtaacattctttgaccttggttagctgctctttgagctttgacatggtcgcaaacatttcttttccttcttcttgggggctttctttggtaatgaggtgtgctgtctttgtaattatcttgtattgggcatccatcacaggcaccctctgctcaatatcctccaagtcttgaattaatagcttgacattcataaaagagacttctaagggttcagaaagtttcttatgggcttccgttgcaaaagcagacagggtaacaacacagtctgtgtattccttcttcattctgtccatctcatcagcttgagcatattgcttgacttccataaacaactccctccaccgcccatttagcaacagtaattgctgcttcaggtcacgggaaaccatctcatcacaggtttcaattagaaaattgccagcatcgttcatggcagtatgctgctgaatccaatgaggtaaatttcgaaaaaaatcctttttggcattttctgattgattgagcattttttcagcatcctctagccaggcttgcagactagccactgtattgccatagcgatcccagttagagatcacttcttccagcatgctcctcacactcctcacttctactgagagattcctccactgagcggtggtttcattcatgaatttcatcacattctcagcttcttccactgaaccatctgctttgacatacatctcagctgtctgtttcaagatctggtatgtcacctcatattgttcaaagaacttgctattttctataaaagacacgtagttttgtagaagctgctccactgactctctcctcccgtacttaatgatccaagacttcagctttgactctgcaagaaccagcagtgagagcagacggtactttaattctaaaaattccattttcattaggtgtagctctgatgtggaggaaacaaaatgaaacctctcggccatgtcctctaattgatcaggtggcactggaatcccgttaacagacctggtccggtagatttcatggaatgctcttttgtgggcatccgtgttttgaagcagatccttatgttgctcaagtttccgttgtatcgtgtttgctgtttcctcgtggacctgttgaacggttatttcctctctcagggccacctccgctctgtacagccaggcacctatggtgcccagaggtgcaggaagagatttatcaagctgtatatgccagtcaaagagcctggaggtcactctatcccaagattgttttaccaatgcttggtcaagtgacaatttaccgtctctgtgtaatggttgtattaaatgttcaatctgtttcctcttcatttcatattgaactctgaagtgcttaaatgactgatatttatcctgtaaatttgattccaccatctgtgctcttgtcaaatctctctcaaattgttctatccaaactttcatttccttaaaaattactctgtcttctctcttaaaattttgtacagaatttgcaaaagatgggaaacctggaagtatttcatcatcctcttgcccatcagtgcttgcattgtggatgtcaggataatgtttcagaaactgggctacataggtcataatagatttctcatctggtttatccacatcaacgtcttcaggatctagcagtcttgggatccccagttctgtttcggcgatagtgaaagcatcctccaaattttctcggttggatctgcctttcactgtctccaagtccaccaattccggtcgaatggcatgaataactgaatgaaaggcaaccccgcttctccaactcttcccaaaatcttttacttctattccagtctgcttgccagctgtgtactgaacccactttaataaagccttcttagcatttccttggatcttggtggtcaccttccgtttacttggtgggctgggagtctcagagctaactatgctgtccacggaggatgcgctgctggacaaagactggagctggggcaggttgctggtcaactcttcaatctggaaatatagaataatggtccacatcaatccaagaactattgagggtcggccatcagctatatcggtggagttaatgttgactaatttaatcggtgatcctctgtgcatggactttcttccttcgaggaacttgagtgccgtgccaatgttagccacagcatggattcgcttcatccggcgtccttgttcacaaggcagtttctgcccagacaggacctccagaagggcaagcagtttaacaccatctttcatgtcttcaaaaagatcgtccaccaccattggaggtttccgcttggccagatgagagttgatccattttgtgaaagttcgtttttgtactatctcttgctcatcttgcagcctctgcatcacattggcgatatcccgaggacaccgggaggcccctctggaggttgccatggtccctccggaagcacgaagccaacaccaagagactcttcactggaggcagcacagggctacaccactctagaaaacatgcttggacttttctagatctattctgtcataaatgaattccaggcctttgcagcactcaacaaggaggcagctctcccaaagactgaactgcttctttttcttcttccgttttaagactgtcctcttacatgaactcaagaaccttctctctcggcctcgttcagtttcccagcagcaaggcgaagcgagcgaacgcttcctcccggctctctgcgcccaggctcggcgggaccccggggatgcgcggctgtccgcccgccctgtcgccgggatcgggcgcggtctgcaggactgcgggagcccagccgccctggtgacagaggacaacaatctcagcccgctgcggccggcggccgcggcccggcgcccgcgctcaccctggctggctcgcccacactcact

SEQ ID NO: 9574 - RNA, 14000 nt, Homo sapiens
  source 1..14000: mol_type = other RNA
agttcttcagtggcaagctttatcaaaatcttccttaaaatgcttcctagaaaccaaattcttctctagttcttgtaaccggtgactgcacttttgtaaaacactgtcatagacactctgcaattcctgaagcttccccagcacttcactcttttcctgctctgtgacttccttcattagttcgcgaccctgggcccaaagtccagtgacttcattttggtaagtcttgaggctggcttgtgcactcttacatgttttgacttgtttgctcacatcatctggtaacagacagatgtgttcacggaacattatctttcgctcatgttgctgaatttggctggtggcctggaacactgccatgagaaactgggttttctcggacaaggctttgtttaagtactttcttcgctggcccactaagtcactgagacaattcacgtggctttgtgcatcagagagagccttctggatgacctgtcgctcattgagaccaagatctgccatgaccctgtctgcgtcctttataagcgatttcaggagcatctgcttggcctccagttcactgcagatggccaggtgatccatgagaaggttctgagccatatctggaggagggctctgcttaagggcctcggcgatgttgggttgttgctcttctgcccactccattagctcctgaaatctggactgcaccacatttaactcctccaagttggtgactgacacttggattttccttttaatgaggtcctcaagctgaaaccaacgttgctctaaatgactcgtctgttctttgactaactccttgtcatctaaattcagatgctctatcattttctgcttttgatctttcagatcttcaatagcatactttctctcctgcaatgccaatgctaactttttcaaagcttccaggtggacagctgtactctctgcatcagatctggccaagttatcccattctgtagtaaatttttctaggaacacttcaacaacattcatacagtcatggtaatctcttgttctctgaagatcctcttccctttgcaagcacaggttgttagactgacggcacaaatcgagccactgatcatttaaatgatttatttccttgtgttcaggcgattcctccttctttgttaacttattcaccttttctattatggtgttcacggatgcctgtttgctctgtagtttcttaacaaaatccttaacttgtgaaaccatgttctgtgcaatgttcagctccagctcagagtgcctcctcttcatgttctgcagttgctgatcagcatcttgcaggtaaatccagagctcagacttcaggtgcttgatctcttcccagccctgagttaagttctgggcctggacaagcttttgttcaatcgtttgctctgtttgttgaatgtcttttgctgtggttttcaccgaagcatttgacaggtcacacatggagcaaaggagatctaggtaggtccttgcctgctcttgcaaagctctgaagtgtttgacctgcttaatggcttctgccctactaagaggtggttgaggacttggctctaaatccggctggactgcagaaagccaggcctggcactgctgcagggtgtcttgtcggctgacgtgcttctgaagttcgtgttccaaactctggtacatcctctgagctgtgctgcagatcgctgagtagctgtcctttgtgccctgcagatgagcatgcacgttttgtttaagtttcgcttgcaggtggtctgcacattggccaatcaaagtatcacctttcatttgaagattgttcaaacggtcttcaaaaccagcaatttcttccatcattgccttgtggtgggccaattgctgggtgattgtctccaggctgcttgtctccaggaggtcaggtgccaccagtctgccagacatctgcagcagccacttttcgacctcttggagctcactgttgtagtcttcatggtctttgactttcgcctccagactgaagacatgctcctttcctatgctgcacaggtcctggtaatcactttgaagttgatctattttgtcctttaaagtgacgtcctgcaccagttccaaaagagcttcacccttctctctcactgactttactgatggttcatgggacagcaccgtttgttgaagtgacttgtatttagataactgagcttttttctcatataattccattttgggttcttcaggaacatgtagaatttcctggtattctgctatccactgtgtcagtgctttgcatttatctgagaattcctttgctaaatgaagacctttttccagcgtcatgtgttctttccggacagtgctggtcagttccttcaactgctccatgtgatcatgaatctcctttcttaacctctctgcctcgccttcctccaagtatttaacagccctctctcctttctcccgggctgatttcagcaaactgtgacctttctccatgtctttgagcaaaacctccaacgtcttcaatttcttccccatcattactgtatctactttgtcaatcttggtagccacattcttgaagtttttatgagtagagccataccaatcagaataggaactgagggatgattctgattcctccaaactctgaatctcctcctccaggaattttatttgttccagcacttggagaagcagggcctggtatctggaagtcagctgggtggcctggcaacccattctgctgttcacgtggctctcgtccagtatctcctgagctctagctcccacttcctcaacttcatctctgtatgcagtcacttcttcgtgccacttcttcatctgatgtaattgtatctccttggttgccctgttagactgacgtctggtcctgggactaactttctcctctgctgttttgagccattcatctacttgctgaaacttttgctccattagcctcaatttgttcaccacgttattgaactgagttcgagtctcggacagcctgtgctggtaagcctgccagtcttgccggagagactctaaagcccggtcctctgcctgtgggatacctgatgggatcacatcctctctggtgtgcagcactgagttcaacagggcctgcccctctgcacagtgtacctgtagctcctgaagatcacgcaatgttgtctcatgagtgtgggcatcaccttcaagaactgaatactggtcgagcttttcttgttcttgccccaaccaaacttcaaatgcctttaggtctctctgatactcttggtgcaggcggacaagtttttcagacttggttacggcttccttggccctctcttggatggctctgtatcgttcctgtagatcctggagttctagctgggtgacatagtgttctgtcatgccagcccctttgacttcgatggtctccagcaagctgctgtaactcagcacttcttcatttaataacttggcttttccgagcatcgttgttttatcccgcagctccgcatgctgcctttctgattcattcaggttggcttccatactatccatccaaccggagaactgtcgaacgccatcctgataacttgtccacttggagagagctccttcgagttggcttttacaacgaatccctgcagacaaaagggatgcccacatatccttcacactctgcagctgctgctgaatagtgggaatgccttctggagaagtattctgaaggacagattctcccctggtcactatcattttcatctgaatctctttttcctgtttgactgataatagagcctcgagcttgagcgtcctgctgtccagcacacttttgtcggatgtcgggtggcagtatgaatccagcatgtgaatcgcatccgtcatccagtcttgtaattctttaatcccaagagagaactgattgtgttctgcaacgattctatccagtcttgacactttctcctttgttaaattgcttagcgctagatactgagaagacagctgcgacactctgtgcctaaagctcttgctggcagcttgtccttcccacagctgctgagctttctctttcagcctgttgagctgaggctcgtagcagtgtatttcctcaaggacagactggagcttctgctgctccctcctctttgctggcagatcatagaggcgattgctgctttcatggaccatcttctcagttttactcagccagtcctggataggctcagcacttacttcaaagtccttcatttggatctttagattctctagagcagattctttttggtggagatttgaatgaaaatttttccaatcttcttttgcagctgtaactttggcctggatccctttcgctttctctttggtcagcagggtactcagaagttcccctttagacagcatcatgtttagcttgtgctgtccattttcactttctgacaaaaactcctgtattttctgaagactagttgaaacttcacttatattttgaggtatatcaaaacacttggcggtagtgatttttgcattaaccaaccactgctggaaatccctgaaggcctttcgaaatctttgctgtaaaatctgttctttattctggcagcccttggatgcttgcaaacaaagacaattatactctttaatcaagccagaaacttttccactgtaggtactcaggtctctggaaaatcgacaaagttcattcagctgagacttgagatcctctgttctaggctctgctttttgcaaagcatccagtatctcttgtcctttgtgccagcattccactatctcctcatccgtgttcttgccttccaggagggttaactgctgagcccaggttttcagaagggcactgaactgttccagggcctgctccagttgagccacttggcctgagaattcctgctccgaaagggccatctggctgaccaggttctccaaacagctctgcgtttggaatacactgtcttcccactgcttccagtcggcacgcagggcctgcatctccgtgtgcatgagctcacacccactggcagttgtgttctgtttcacttcgggagccagcgactccactctgctgagacggcttgcaccaatctctctggaatctatcagctccttaatttttgataactttttctgggtggctgatgaatctccagacatatctgaccaccggtgaagttcttcctttgctgaatggagccaatctgtgaactcgtggaccgcatctaaatacattagatgatctttcacaatctcttccactttcctcattttttccttggcaacagtcattatatcattaaactgtgttttcagctcctcttgagctgtgtccttgaaagactcatcctctgtcttttcgtagagctccctggacttcgcaattagacggtgaagggctctcgtgtgatcttctgcctcagacaggatggactggaggtggtcaagcaggacgaacttctctttcagacctggctgtggttgtaagggatgttctattttttgatccactgattccatccactgctccaactggtttttcctctctacatagtcattccattggctaatcacagactctaaagtgctttgagcgtggacggaggagctcatgatgtcagcccacacttctttaagggtctctaactgagtctgaatcaccctctgaccttctttgttgctacttctcaaggcctgttcccccttgccaatggccatattcaacttaacttccccttcacctttcatcaggagaatatcctgtatttgtgacagccgtttctccagggtgtctttgctcccaagagtgctctctgcacaggccagtctgtcctgaatggccttcacccagaaccacatgctttgcagtgcttcctccagggcttcgtgctcctgaagggccacctggcagctccggagtttctctttggtcattctaagtaggttctggtggcttgtgaggagctgggaacacaggcggccctcctgcccagcaccgtggccttcttcactcagaagctgccctctctgggaaagcttatcaagagactctcttgcagccagcagttctcccaaaaacatttcaactttatgaacttcatttttcttctcaggaatgtgctgtttactctctcccaagttttccgtattgaacctttcttccatttcatggatccataagttcagttttctgtgctgatcttcaaagcttccaagttctgaagcacagtcttgaagagcctgcttatctttaaggcattgtttcagaaatgcttgaaactcttcattggcctttgtgatttgttcttgaatgctactgacaatttgtttagacaaatgtgcatacaaagtttgtccttcttgagtcactgcatcaagtttgctctgcccatcactgactgagtccaaaatgttctgaagatcatggagctttgcttctagaactttgctgtcaccggtgcgatctgatgattcttttgctgctgcctttgctcccaaaaaccattcttggaattcctgcatagactcactgaagtgtttttccagagattcctgcaggctggcctgggttttggagcacaactggctcacggcttcatgtttctttatcagaccagtcattgcacggcccaggctctccaactcagctgagtggtacttgcggcacaagctattgagattttcttgggtagagctgatgttgctttgttgactttgaagttctttttgtatatccttgacttttttcaatgcttcacaagtctcattttgggcacagttcatcaacgattcttccacttttgtgaaccatgttgttatgtcattaataaacttctccacttgtgtactttgagccgtgaaatccttcagggttccttttgctacttcagttatttctttggcatgctccagtttctgcattaagtctgcttctataaactgaaggtctggcggtgtttctagatttttagttaattctttcagatcattaactttggaatgcagttcttccaatctcaatgctttgtttttaacttcagactcaaattctttaagcagttcttcagctctgaggtggttatccaggttgctgatgttttctgccatctgtggaacgcagttgtttgaccatccctcaatctcatctctagttgacagtacatcatcccaaatggacaggcttactctcagcctatccatgttttcttcaagtttctctgatacatccagccatttgtccacggtgctctccatgtctgttttcaccaagctgaaatcactactgtgaattttcttcagctcagataacaagtgttttcctttgctggtaaagttatccaagtctttctgtttgtaattcattttgttcttggcagtttcatgcttggaaaaagcccatttaagatcctcctgatcttttatggtagttctggttacaatcacactgctggcattttctaagactttagatacagctgatttcaggttctgatattctctcattaagtcaataagtccacagcactgaccctgattttcatgaattagtcttttggtatcatcccaggtgacctctaagcggtttatctccctgtcaacttcaggtgcaaaagctacatctttctgggcaatttgcttggctttgtctttcaaccaacatagttcatgctcgtgagaattcaattcatcttctagctgattaaacactcttaacctctgctgaagagcttggcgggtaggttctttcaatcgctctttgtcagtcctttcttcaatgtcctcaatgcttttcagaagctcctctttctggtcttggaatgcttttttcaacactgccagagcatctgcctcactctgcttggttcccagaaggttctggatcctctctacctctccacagagctgatcagccgtggctctgcaggaagtcctttgctcagagctcccgattttcagatggtattgggctttggaaagaatgccatccagactgacggcagcagattctaatgctttagcattttgaagagcatcattgaggtccttttctatcaaatcagactcgttcttattcatactgttggttgcttccactgtttgcctcagctggcggagaatgccggacagagaggcatggctctggaggaattctgccaaatgggacagggcaagctgccgcctctccacaacctggctggcctcctcaaacagctggaagcagtcctcagcctttccctgcaggaggtggaggtcctcagcacggcccagagaacccaactttgctaagtgaccctgcagactctgcaattcgccctttttgctctctacttctgctgcgtggtccttatgccgagtaagggctacttgatggtccattatgctaatctcagaggtagtttgtaattcactgagaaacagtttaatccagacagaaaaggaaagcagcagctcatcaaattgctggtgttcagcaaccacagactgaagaaaattaatccttttgttaatgatctgtggtaaatctctccatctctcatccaactgctccaaatgtagtttcatcattttcacatcatctttggaggctactgagaacaatgattccttcaattgcaaaagtttgctatagaatgaggcctgggatacaacttcattttgcagtgcctgtattaactgaagttcaccttccactttgactctgtctgcagaaatgtccatttctggggaactggctttagcttcaccccgctctaaccaggtcaaaaaggatgatagttctttctctagcctctgccagtgggccagcagattctccagcgccgtctgtctctccttcgccctccttaggatgtcctcgtattgctgctgtagagccgcagcctcctgaacacaggaatctctgttcacaaccttcctggcactggctgagaaggcagtgatcgcgctgctcagtgactccagggcctggcagagatccatatgttcttgaagaactttgtatgtttctgtagctgaagaacatattttaattggaacagcaagtttatcttcaaattcagacacagattgctggatctttctaaggttctcttcaaacttttgctgctgagataaatgtcccaggattgttccttccagacactgtgcatgctctcgaagctcttccccgtatcttcttatttgtgtcaacttggctttaattcgagcagattctccagtggtaacaaactgagcaaaagactgggcttcttcttctaatcctacaatgctgctgagcttactttctatttcctgaattgtgaccttaatttggctgatttgcatgtccatggcagatgacgaagtttccaaggcattgagttctttttctttctcagttatccagacggacagagtctcaaaattactgccaaaatgatcccacttggttttcaccatttccatggttttaatatcttcttcaagcgtgtcttctaattttttgacttgttctttgattgacttggcctgctgttgaagcagctgcttattttggggcccaagcggtatctctgaagcttcctttacaaggttctcagcctggactgcaatactttctgtccgtttagaaaactcctttgtttgttccagttctgaagataaactttccaaactgctaaaactcaagaagcgttcatgactggaacctgtttgaaaaaggtatcttactactgtttctttgtttgtttcaaatcgctcccattttcttaatgtgacctggatgcggcgttcctgcctctcccggctgcgctccaggccatccagtgtgctctccagcttccgcagctcctcgtggcctcggtcaggcagccccccttctccctgctgcgcctgcgcgatctgctgctgcacatctctcttctttgctgagatccgctttgtcttttgctggtgatgaagaagtaactgctgtgcttcaaacagattttcagtatccaagatcttctcagcttgttcctggacttctttagagccagaaattaattcttcgagagaatttttgactatttctttgtactggacacagtccccaaaattgcttagcatcttttcaacctctgacagcagcgtcacaagagccttgaaagagctggataattttgccagctcatctccctgcttttgggcttcattctcagaagaaacttctgtcaaaactttcagcctggatttcagccagctgagggtctcaccccttttggtaacaccatttctgatctcttcaacggcacgtttaacctctccgtggttggcagtatcgatggcctcacccttgatcccctttaattgtgtctcatttgtagatatccaagatgagaactcagagaatctgctagtgtagtccttccacttgtctgggtcttccatgagcttcctgtaggtgctgtcaatggcagctctgagctctttgagagtcacgtgacaggttccaggtgtgtcccttactgggtcccgcactgggagtttcacacagagttcctcgatgagctgtaaccttttctcacagagatgatgaggacctttgtcactgaagaaaaccctgtgctctttaattatcttttcactgccttcctggggcatcagcttggtctctcgatccagctcagttctgcattcttctacagaggctaagaacctattcttctccacatcaatcttcagatgaagcaaatgataaggggcttctccttgaagatccttccattgtttgtggagctttcgaacagcttcctgcagcccctgctgctcctgctctggaaggatgtcggtgagttcatcacaagctttcaggaaagcattgagcaccctctgatccagctgactgaaaaactcagtgtgtctccgcaggagctcctctggatcccccttttcctccaggccctcctgagcaatccgcagtaccttctccaactctgctcgagactcctcaaacttcttcatcaagcgactgttggtttccacatgcttcttccaatctccagttttctttaccatactctgaaaagcaacatgaatatctgcaatctgtctttgtagcctcgtctgatcaaaatgctttaacacgttgctcaaggtcacaaacttttgaacactttgactgcctttctcaataagtgtcaaggttttcttacagttttcttgacaagctaacagttcctgatgtttttgtttaaaaagggcactcgattgtgcctcacgctcaagaactgtgataatttcattgattttcccaagtgagtcataaaaggacgtcatctgcttttctaattcctccaacggaatcaacagctgctgagactcataaaggagtggggagtaacattctttgaccttggttagctgctctttgagctttgacatggtcgcaaacatttcttttccttcttcttgggggctttctttggtaatgaggtgtgctgtctttgtaattatcttgtattgggcatccatcacaggcaccctctgctcaatatcctccaagtcttgaattaatagcttgacattcataaaagagacttctaagggttcagaaagtttcttatgggcttccgttgcaaaagcagacagggtaacaacacagtctgtgtattccttcttcattctgtccatctcatcagcttgagcatattgcttgacttccataaacaactccctccaccgcccatttagcaacagtaattgctgcttcaggtcacgggaaaccatctcatcacaggtttcaattagaaaattgccagcatcgttcatggcagtatgctgctgaatccaatgaggtaaatttcgaaaaaaatcctttttggcattttctgattgattgagcattttttcagcatcctctagccaggcttgcagactagccactgtattgccatagcgatcccagttagagatcacttcttccagcatgctcctcacactcctcacttctactgagagattcctccactgagcggtggtttcattcatgaatttcatcacattctcagcttcttccactgaaccatctgctttgacatacatctcagctgtctgtttcaagatctggtatgtcacctcatattgttcaaagaacttgctattttctataaaagacacgtagttttgtagaagctgctccactgactctctcctcccgtacttaatgatccaagacttcagctttgactctgcaagaaccagcagtgagagcagacggtactttaattctaaaaattccattttcattaggtgtagctctgatgtggaggaaacaaaatgaaacctctcggccatgtcctctaattgatcaggtggcactggaatcccgttaacagacctggtccggtagatttcatggaatgctcttttgtgggcatccgtgttttgaagcagatccttatgttgctcaagtttccgttgtatcgtgtttgctgtttcctcgtggacctgttgaacggttatttcctctctcagggccacctccgctctgtacagccaggcacctatggtgcccagaggtgcaggaagagatttatcaagctgtatatgccagtcaaagagcctggaggtcactctatcccaagattgttttaccaatgcttggtcaagtgacaatttaccgtctctgtgtaatggttgtattaaatgttcaatctgtttcctcttcatttcatattgaactctgaagtgcttaaatgactgatatttatcctgtaaatttgattccaccatctgtgctcttgtcaaatctctctcaaattgttctatccaaactttcatttccttaaaaattactctgtcttctctcttaaaattttgtacagaatttgcaaaagatgggaaacctggaagtatttcatcatcctcttgcccatcagtgcttgcattgtggatgtcaggataatgtttcagaaactgggctacataggtcataatagatttctcatctggtttatccacatcaacgtcttcaggatctagcagtcttgggatccccagttctgtttcggcgatagtgaaagcatcctccaaattttctcggttggatctgcctttcactgtctccaagtccaccaattccggtcgaatggcatgaataactgaatgaaaggcaaccccgcttctccaactcttcccaaaatcttttacttctattccagtctgcttgccagctgtgtactgaacccactttaataaagccttcttagcatttccttggatcttggtggtcaccttccgtttacttggtgggctgggagtctcagagctaactatgctgtccacggaggatgcgctgctggacaaagactggagctggggcaggttgctggtcaactcttcaatctggaaatatagaataatggtccacatcaatccaagaactattgagggtcggccatcagctatatcggtggagttaatgttgactaatttaatcggtgatcctctgtgcatggactttcttccttcgaggaacttgagtgccgtgccaatgttagccacagcatggattcgcttcatccggcgtccttgttcacaaggcagtttctgcccagacaggacctccagaagggcaagcagtttaacaccatctttcatgtcttcaaaaagatcgtccaccaccattggaggtttccgcttggccagatgagagttgatccattttgtgaaagttcgtttttgtactatctcttgctcatcttttatcatacccggagtcttgtagattgtttttatcatatctcacctattttactgattttggtaaattatcctaattcagtcgtatctaaaccaaacacagctttcaccaagggaacttccaactctcctagcagcattctcctgatattatcactatagcaacatctctataaaagcatactattcttccctcattcttcatccttaccccctgcttactagccaaatgcaccgctccccagtgccagcgtgtctacaaagacagtgctcatatcgatttataaaaagtgcttcagatgcacttt

SEQ ID NO: 9575 - RNA, 14142 nt, Homo sapiens
  source 1..14142: mol_type = other RNA
agttcttcagtggcaagctttatcaaaatcttccttaaaatgcttcctagaaaccaaattcttctctagttcttgtaaccggtgactgcacttttgtaaaacactgtcatagacactctgcaattcctgaagcttccccagcacttcactcttttcctgctctgtgacttccttcattagttcgcgaccctgggcccaaagtccagtgacttcattttggtaagtcttgaggctggcttgtgcactcttacatgttttgacttgtttgctcacatcatctggtaacagacagatgtgttcacggaacattatctttcgctcatgttgctgaatttggctggtggcctggaacactgccatgagaaactgggttttctcggacaaggctttgtttaagtactttcttcgctggcccactaagtcactgagacaattcacgtggctttgtgcatcagagagagccttctggatgacctgtcgctcattgagaccaagatctgccatgaccctgtctgcgtcctttataagcgatttcaggagcatctgcttggcctccagttcactgcagatggccaggtgatccatgagaaggttctgagccatatctggaggagggctctgcttaagggcctcggcgatgttgggttgttgctcttctgcccactccattagctcctgaaatctggactgcaccacatttaactcctccaagttggtgactgacacttggattttccttttaatgaggtcctcaagctgaaaccaacgttgctctaaatgactcgtctgttctttgactaactccttgtcatctaaattcagatgctctatcattttctgcttttgatctttcagatcttcaatagcatactttctctcctgcaatgccaatgctaactttttcaaagcttccaggtggacagctgtactctctgcatcagatctggccaagttatcccattctgtagtaaatttttctaggaacacttcaacaacattcatacagtcatggtaatctcttgttctctgaagatcctcttccctttgcaagcacaggttgttagactgacggcacaaatcgagccactgatcatttaaatgatttatttccttgtgttcaggcgattcctccttctttgttaacttattcaccttttctattatggtgttcacggatgcctgtttgctctgtagtttcttaacaaaatccttaacttgtgaaaccatgttctgtgcaatgttcagctccagctcagagtgcctcctcttcatgttctgcagttgctgatcagcatcttgcaggtaaatccagagctcagacttcaggtgcttgatctcttcccagccctgagttaagttctgggcctggacaagcttttgttcaatcgtttgctctgtttgttgaatgtcttttgctgtggttttcaccgaagcatttgacaggtcacacatggagcaaaggagatctaggtaggtccttgcctgctcttgcaaagctctgaagtgtttgacctgcttaatggcttctgccctactaagaggtggttgaggacttggctctaaatccggctggactgcagaaagccaggcctggcactgctgcagggtgtcttgtcggctgacgtgcttctgaagttcgtgttccaaactctggtacatcctctgagctgtgctgcagatcgctgagtagctgtcctttgtgccctgcagatgagcatgcacgttttgtttaagtttcgcttgcaggtggtctgcacattggccaatcaaagtatcacctttcatttgaagattgttcaaacggtcttcaaaaccagcaatttcttccatcattgccttgtggtgggccaattgctgggtgattgtctccaggctgcttgtctccaggaggtcaggtgccaccagtctgccagacatctgcagcagccacttttcgacctcttggagctcactgttgtagtcttcatggtctttgactttcgcctccagactgaagacatgctcctttcctatgctgcacaggtcctggtaatcactttgaagttgatctattttgtcctttaaagtgacgtcctgcaccagttccaaaagagcttcacccttctctctcactgactttactgatggttcatgggacagcaccgtttgttgaagtgacttgtatttagataactgagcttttttctcatataattccattttgggttcttcaggaacatgtagaatttcctggtattctgctatccactgtgtcagtgctttgcatttatctgagaattcctttgctaaatgaagacctttttccagcgtcatgtgttctttccggacagtgctggtcagttccttcaactgctccatgtgatcatgaatctcctttcttaacctctctgcctcgccttcctccaagtatttaacagccctctctcctttctcccgggctgatttcagcaaactgtgacctttctccatgtctttgagcaaaacctccaacgtcttcaatttcttccccatcattactgtatctactttgtcaatcttggtagccacattcttgaagtttttatgagtagagccataccaatcagaataggaactgagggatgattctgattcctccaaactctgaatctcctcctccaggaattttatttgttccagcacttggagaagcagggcctggtatctggaagtcagctgggtggcctggcaacccattctgctgttcacgtggctctcgtccagtatctcctgagctctagctcccacttcctcaacttcatctctgtatgcagtcacttcttcgtgccacttcttcatctgatgtaattgtatctccttggttgccctgttagactgacgtctggtcctgggactaactttctcctctgctgttttgagccattcatctacttgctgaaacttttgctccattagcctcaatttgttcaccacgttattgaactgagttcgagtctcggacagcctgtgctggtaagcctgccagtcttgccggagagactctaaagcccggtcctctgcctgtgggatacctgatgggatcacatcctctctggtgtgcagcactgagttcaacagggcctgcccctctgcacagtgtacctgtagctcctgaagatcacgcaatgttgtctcatgagtgtgggcatcaccttcaagaactgaatactggtcgagcttttcttgttcttgccccaaccaaacttcaaatgcctttaggtctctctgatactcttggtgcaggcggacaagtttttcagacttggttacggcttccttggccctctcttggatggctctgtatcgttcctgtagatcctggagttctagctgggtgacatagtgttctgtcatgccagcccctttgacttcgatggtctccagcaagctgctgtaactcagcacttcttcatttaataacttggcttttccgagcatcgttgttttatcccgcagctccgcatgctgcctttctgattcattcaggttggcttccatactatccatccaaccggagaactgtcgaacgccatcctgataacttgtccacttggagagagctccttcgagttggcttttacaacgaatccctgcagacaaaagggatgcccacatatccttcacactctgcagctgctgctgaatagtgggaatgccttctggagaagtattctgaaggacagattctcccctggtcactatcattttcatctgaatctctttttcctgtttgactgataatagagcctcgagcttgagcgtcctgctgtccagcacacttttgtcggatgtcgggtggcagtatgaatccagcatgtgaatcgcatccgtcatccagtcttgtaattctttaatcccaagagagaactgattgtgttctgcaacgattctatccagtcttgacactttctcctttgttaaattgcttagcgctagatactgagaagacagctgcgacactctgtgcctaaagctcttgctggcagcttgtccttcccacagctgctgagctttctctttcagcctgttgagctgaggctcgtagcagtgtatttcctcaaggacagactggagcttctgctgctccctcctctttgctggcagatcatagaggcgattgctgctttcatggaccatcttctcagttttactcagccagtcctggataggctcagcacttacttcaaagtccttcatttggatctttagattctctagagcagattctttttggtggagatttgaatgaaaatttttccaatcttcttttgcagctgtaactttggcctggatccctttcgctttctctttggtcagcagggtactcagaagttcccctttagacagcatcatgtttagcttgtgctgtccattttcactttctgacaaaaactcctgtattttctgaagactagttgaaacttcacttatattttgaggtatatcaaaacacttggcggtagtgatttttgcattaaccaaccactgctggaaatccctgaaggcctttcgaaatctttgctgtaaaatctgttctttattctggcagcccttggatgcttgcaaacaaagacaattatactctttaatcaagccagaaacttttccactgtaggtactcaggtctctggaaaatcgacaaagttcattcagctgagacttgagatcctctgttctaggctctgctttttgcaaagcatccagtatctcttgtcctttgtgccagcattccactatctcctcatccgtgttcttgccttccaggagggttaactgctgagcccaggttttcagaagggcactgaactgttccagggcctgctccagttgagccacttggcctgagaattcctgctccgaaagggccatctggctgaccaggttctccaaacagctctgcgtttggaatacactgtcttcccactgcttccagtcggcacgcagggcctgcatctccgtgtgcatgagctcacacccactggcagttgtgttctgtttcacttcgggagccagcgactccactctgctgagacggcttgcaccaatctctctggaatctatcagctccttaatttttgataactttttctgggtggctgatgaatctccagacatatctgaccaccggtgaagttcttcctttgctgaatggagccaatctgtgaactcgtggaccgcatctaaatacattagatgatctttcacaatctcttccactttcctcattttttccttggcaacagtcattatatcattaaactgtgttttcagctcctcttgagctgtgtccttgaaagactcatcctctgtcttttcgtagagctccctggacttcgcaattagacggtgaagggctctcgtgtgatcttctgcctcagacaggatggactggaggtggtcaagcaggacgaacttctctttcagacctggctgtggttgtaagggatgttctattttttgatccactgattccatccactgctccaactggtttttcctctctacatagtcattccattggctaatcacagactctaaagtgctttgagcgtggacggaggagctcatgatgtcagcccacacttctttaagggtctctaactgagtctgaatcaccctctgaccttctttgttgctacttctcaaggcctgttcccccttgccaatggccatattcaacttaacttccccttcacctttcatcaggagaatatcctgtatttgtgacagccgtttctccagggtgtctttgctcccaagagtgctctctgcacaggccagtctgtcctgaatggccttcacccagaaccacatgctttgcagtgcttcctccagggcttcgtgctcctgaagggccacctggcagctccggagtttctctttggtcattctaagtaggttctggtggcttgtgaggagctgggaacacaggcggccctcctgcccagcaccgtggccttcttcactcagaagctgccctctctgggaaagcttatcaagagactctcttgcagccagcagttctcccaaaaacatttcaactttatgaacttcatttttcttctcaggaatgtgctgtttactctctcccaagttttccgtattgaacctttcttccatttcatggatccataagttcagttttctgtgctgatcttcaaagcttccaagttctgaagcacagtcttgaagagcctgcttatctttaaggcattgtttcagaaatgcttgaaactcttcattggcctttgtgatttgttcttgaatgctactgacaatttgtttagacaaatgtgcatacaaagtttgtccttcttgagtcactgcatcaagtttgctctgcccatcactgactgagtccaaaatgttctgaagatcatggagctttgcttctagaactttgctgtcaccggtgcgatctgatgattcttttgctgctgcctttgctcccaaaaaccattcttggaattcctgcatagactcactgaagtgtttttccagagattcctgcaggctggcctgggttttggagcacaactggctcacggcttcatgtttctttatcagaccagtcattgcacggcccaggctctccaactcagctgagtggtacttgcggcacaagctattgagattttcttgggtagagctgatgttgctttgttgactttgaagttctttttgtatatccttgacttttttcaatgcttcacaagtctcattttgggcacagttcatcaacgattcttccacttttgtgaaccatgttgttatgtcattaataaacttctccacttgtgtactttgagccgtgaaatccttcagggttccttttgctacttcagttatttctttggcatgctccagtttctgcattaagtctgcttctataaactgaaggtctggcggtgtttctagatttttagttaattctttcagatcattaactttggaatgcagttcttccaatctcaatgctttgtttttaacttcagactcaaattctttaagcagttcttcagctctgaggtggttatccaggttgctgatgttttctgccatctgtggaacgcagttgtttgaccatccctcaatctcatctctagttgacagtacatcatcccaaatggacaggcttactctcagcctatccatgttttcttcaagtttctctgatacatccagccatttgtccacggtgctctccatgtctgttttcaccaagctgaaatcactactgtgaattttcttcagctcagataacaagtgttttcctttgctggtaaagttatccaagtctttctgtttgtaattcattttgttcttggcagtttcatgcttggaaaaagcccatttaagatcctcctgatcttttatggtagttctggttacaatcacactgctggcattttctaagactttagatacagctgatttcaggttctgatattctctcattaagtcaataagtccacagcactgaccctgattttcatgaattagtcttttggtatcatcccaggtgacctctaagcggtttatctccctgtcaacttcaggtgcaaaagctacatctttctgggcaatttgcttggctttgtctttcaaccaacatagttcatgctcgtgagaattcaattcatcttctagctgattaaacactcttaacctctgctgaagagcttggcgggtaggttctttcaatcgctctttgtcagtcctttcttcaatgtcctcaatgcttttcagaagctcctctttctggtcttggaatgcttttttcaacactgccagagcatctgcctcactctgcttggttcccagaaggttctggatcctctctacctctccacagagctgatcagccgtggctctgcaggaagtcctttgctcagagctcccgattttcagatggtattgggctttggaaagaatgccatccagactgacggcagcagattctaatgctttagcattttgaagagcatcattgaggtccttttctatcaaatcagactcgttcttattcatactgttggttgcttccactgtttgcctcagctggcggagaatgccggacagagaggcatggctctggaggaattctgccaaatgggacagggcaagctgccgcctctccacaacctggctggcctcctcaaacagctggaagcagtcctcagcctttccctgcaggaggtggaggtcctcagcacggcccagagaacccaactttgctaagtgaccctgcagactctgcaattcgccctttttgctctctacttctgctgcgtggtccttatgccgagtaagggctacttgatggtccattatgctaatctcagaggtagtttgtaattcactgagaaacagtttaatccagacagaaaaggaaagcagcagctcatcaaattgctggtgttcagcaaccacagactgaagaaaattaatccttttgttaatgatctgtggtaaatctctccatctctcatccaactgctccaaatgtagtttcatcattttcacatcatctttggaggctactgagaacaatgattccttcaattgcaaaagtttgctatagaatgaggcctgggatacaacttcattttgcagtgcctgtattaactgaagttcaccttccactttgactctgtctgcagaaatgtccatttctggggaactggctttagcttcaccccgctctaaccaggtcaaaaaggatgatagttctttctctagcctctgccagtgggccagcagattctccagcgccgtctgtctctccttcgccctccttaggatgtcctcgtattgctgctgtagagccgcagcctcctgaacacaggaatctctgttcacaaccttcctggcactggctgagaaggcagtgatcgcgctgctcagtgactccagggcctggcagagatccatatgttcttgaagaactttgtatgtttctgtagctgaagaacatattttaattggaacagcaagtttatcttcaaattcagacacagattgctggatctttctaaggttctcttcaaacttttgctgctgagataaatgtcccaggattgttccttccagacactgtgcatgctctcgaagctcttccccgtatcttcttatttgtgtcaacttggctttaattcgagcagattctccagtggtaacaaactgagcaaaagactgggcttcttcttctaatcctacaatgctgctgagcttactttctatttcctgaattgtgaccttaatttggctgatttgcatgtccatggcagatgacgaagtttccaaggcattgagttctttttctttctcagttatccagacggacagagtctcaaaattactgccaaaatgatcccacttggttttcaccatttccatggttttaatatcttcttcaagcgtgtcttctaattttttgacttgttctttgattgacttggcctgctgttgaagcagctgcttattttggggcccaagcggtatctctgaagcttcctttacaaggttctcagcctggactgcaatactttctgtccgtttagaaaactcctttgtttgttccagttctgaagataaactttccaaactgctaaaactcaagaagcgttcatgactggaacctgtttgaaaaaggtatcttactactgtttctttgtttgtttcaaatcgctcccattttcttaatgtgacctggatgcggcgttcctgcctctcccggctgcgctccaggccatccagtgtgctctccagcttccgcagctcctcgtggcctcggtcaggcagccccccttctccctgctgcgcctgcgcgatctgctgctgcacatctctcttctttgctgagatccgctttgtcttttgctggtgatgaagaagtaactgctgtgcttcaaacagattttcagtatccaagatcttctcagcttgttcctggacttctttagagccagaaattaattcttcgagagaatttttgactatttctttgtactggacacagtccccaaaattgcttagcatcttttcaacctctgacagcagcgtcacaagagccttgaaagagctggataattttgccagctcatctccctgcttttgggcttcattctcagaagaaacttctgtcaaaactttcagcctggatttcagccagctgagggtctcaccccttttggtaacaccatttctgatctcttcaacggcacgtttaacctctccgtggttggcagtatcgatggcctcacccttgatcccctttaattgtgtctcatttgtagatatccaagatgagaactcagagaatctgctagtgtagtccttccacttgtctgggtcttccatgagcttcctgtaggtgctgtcaatggcagctctgagctctttgagagtcacgtgacaggttccaggtgtgtcccttactgggtcccgcactgggagtttcacacagagttcctcgatgagctgtaaccttttctcacagagatgatgaggacctttgtcactgaagaaaaccctgtgctctttaattatcttttcactgccttcctggggcatcagcttggtctctcgatccagctcagttctgcattcttctacagaggctaagaacctattcttctccacatcaatcttcagatgaagcaaatgataaggggcttctccttgaagatccttccattgtttgtggagctttcgaacagcttcctgcagcccctgctgctcctgctctggaaggatgtcggtgagttcatcacaagctttcaggaaagcattgagcaccctctgatccagctgactgaaaaactcagtgtgtctccgcaggagctcctctggatcccccttttcctccaggccctcctgagcaatccgcagtaccttctccaactctgctcgagactcctcaaacttcttcatcaagcgactgttggtttccacatgcttcttccaatctccagttttctttaccatactctgaaaagcaacatgaatatctgcaatctgtctttgtagcctcgtctgatcaaaatgctttaacacgttgctcaaggtcacaaacttttgaacactttgactgcctttctcaataagtgtcaaggttttcttacagttttcttgacaagctaacagttcctgatgtttttgtttaaaaagggcactcgattgtgcctcacgctcaagaactgtgataatttcattgattttcccaagtgagtcataaaaggacgtcatctgcttttctaattcctccaacggaatcaacagctgctgagactcataaaggagtggggagtaacattctttgaccttggttagctgctctttgagctttgacatggtcgcaaacatttcttttccttcttcttgggggctttctttggtaatgaggtgtgctgtctttgtaattatcttgtattgggcatccatcacaggcaccctctgctcaatatcctccaagtcttgaattaatagcttgacattcataaaagagacttctaagggttcagaaagtttcttatgggcttccgttgcaaaagcagacagggtaacaacacagtctgtgtattccttcttcattctgtccatctcatcagcttgagcatattgcttgacttccataaacaactccctccaccgcccatttagcaacagtaattgctgcttcaggtcacgggaaaccatctcatcacaggtttcaattagaaaattgccagcatcgttcatggcagtatgctgctgaatccaatgaggtaaatttcgaaaaaaatcctttttggcattttctgattgattgagcattttttcagcatcctctagccaggcttgcagactagccactgtattgccatagcgatcccagttagagatcacttcttccagcatgctcctcacactcctcacttctactgagagattcctccactgagcggtggtttcattcatgaatttcatcacattctcagcttcttccactgaaccatctgctttgacatacatctcagctgtctgtttcaagatctggtatgtcacctcatattgttcaaagaacttgctattttctataaaagacacgtagttttgtagaagctgctccactgactctctcctcccgtacttaatgatccaagacttcagctttgactctgcaagaaccagcagtgagagcagacggtactttaattctaaaaattccattttcattaggtgtagctctgatgtggaggaaacaaaatgaaacctctcggccatgtcctctaattgatcaggtggcactggaatcccgttaacagacctggtccggtagatttcatggaatgctcttttgtgggcatccgtgttttgaagcagatccttatgttgctcaagtttccgttgtatcgtgtttgctgtttcctcgtggacctgttgaacggttatttcctctctcagggccacctccgctctgtacagccaggcacctatggtgcccagaggtgcaggaagagatttatcaagctgtatatgccagtcaaagagcctggaggtcactctatcccaagattgttttaccaatgcttggtcaagtgacaatttaccgtctctgtgtaatggttgtattaaatgttcaatctgtttcctcttcatttcatattgaactctgaagtgcttaaatgactgatatttatcctgtaaatttgattccaccatctgtgctcttgtcaaatctctctcaaattgttctatccaaactttcatttccttaaaaattactctgtcttctctcttaaaattttgtacagaatttgcaaaagatgggaaacctggaagtatttcatcatcctcttgcccatcagtgcttgcattgtggatgtcaggataatgtttcagaaactgggctacataggtcataatagatttctcatctggtttatccacatcaacgtcttcaggatctagcagtcttgggatccccagttctgtttcggcgatagtgaaagcatcctccaaattttctcggttggatctgcctttcactgtctccaagtccaccaattccggtcgaatggcatgaataactgaatgaaaggcaaccccgcttctccaactcttcccaaaatcttttacttctattccagtctgcttgccagctgtgtactgaacccactttaataaagccttcttagcatttccttggatcttggtggtcaccttccgtttacttggtgggctgggagtctcagagctaactatgctgtccacggaggatgcgctgctggacaaagactggagctggggcaggttgctggtcaactcttcaatctggaaatatagaataatggtccacatcaatccaagaactattgagggtcggccatcagctatatcggtggagttaatgttgactaatttaatctttcttccttcgaggaacttgagtgccgtgccaatgttagccacagcatggattcgcttcatccggcgtccttgttcacaaggcagtttctgcccagacaggacctccagaagggcaagcagtttaacaccatctttcatgtcttcaaaaagatcgtccaccaccattggaggtttccgcttggccagatgagagttgatccattttgtgaaagttcgtttttgtactatctcttgctcatcttgcagcctctgcatcacattggcgatatcccgaggacaccgggaggcccctctggaggttgccatggtccctccggaagcacgaagccaacaccaagagactcttcactggaggcagcacagggctacaccactctagaaaacatgcttggacttttctagatctattctgtcataaatgaattccaggcctttgcagcactcaacaaggaggcagctctcccaaagactgaactgcttctttttcttcttccgttttaagactgtcctcttacatgaactcaagaacctcctggagatgcacggccttgggcgtttctccgcagctgcaaagctgtgctgtgacccacccgctcagcgagcctttataccgggaccacctcccgggggtcgaggtgggaaggaaatgtccctgagagccgggacgcgctgcctccgctgcctggaggagctgcgctgtcctgccagcta

SEQ ID NO: 9576 - RNA, 14302 nt, Homo sapiens
  source 1..14302: mol_type = other RNA
agttcttcagtggcaagctttatcaaaatcttccttaaaatgcttcctagaaaccaaattcttctctagttcttgtaaccggtgactgcacttttgtaaaacactgtcatagacactctgcaattcctgaagcttccccagcacttcactcttttcctgctctgtgacttccttcattagttcgcgaccctgggcccaaagtccagtgacttcattttggtaagtcttgaggctggcttgtgcactcttacatgttttgacttgtttgctcacatcatctggtaacagacagatgtgttcacggaacattatctttcgctcatgttgctgaatttggctggtggcctggaacactgccatgagaaactgggttttctcggacaaggctttgtttaagtactttcttcgctggcccactaagtcactgagacaattcacgtggctttgtgcatcagagagagccttctggatgacctgtcgctcattgagaccaagatctgccatgaccctgtctgcgtcctttataagcgatttcaggagcatctgcttggcctccagttcactgcagatggccaggtgatccatgagaaggttctgagccatatctggaggagggctctgcttaagggcctcggcgatgttgggttgttgctcttctgcccactccattagctcctgaaatctggactgcaccacatttaactcctccaagttggtgactgacacttggattttccttttaatgaggtcctcaagctgaaaccaacgttgctctaaatgactcgtctgttctttgactaactccttgtcatctaaattcagatgctctatcattttctgcttttgatctttcagatcttcaatagcatactttctctcctgcaatgccaatgctaactttttcaaagcttccaggtggacagctgtactctctgcatcagatctggccaagttatcccattctgtagtaaatttttctaggaacacttcaacaacattcatacagtcatggtaatctcttgttctctgaagatcctcttccctttgcaagcacaggttgttagactgacggcacaaatcgagccactgatcatttaaatgatttatttccttgtgttcaggcgattcctccttctttgttaacttattcaccttttctattatggtgttcacggatgcctgtttgctctgtagtttcttaacaaaatccttaacttgtgaaaccatgttctgtgcaatgttcagctccagctcagagtgcctcctcttcatgttctgcagttgctgatcagcatcttgcaggtaaatccagagctcagacttcaggtgcttgatctcttcccagccctgagttaagttctgggcctggacaagcttttgttcaatcgtttgctctgtttgttgaatgtcttttgctgtggttttcaccgaagcatttgacaggtcacacatggagcaaaggagatctaggtaggtccttgcctgctcttgcaaagctctgaagtgtttgacctgcttaatggcttctgccctactaagaggtggttgaggacttggctctaaatccggctggactgcagaaagccaggcctggcactgctgcagggtgtcttgtcggctgacgtgcttctgaagttcgtgttccaaactctggtacatcctctgagctgtgctgcagatcgctgagtagctgtcctttgtgccctgcagatgagcatgcacgttttgtttaagtttcgcttgcaggtggtctgcacattggccaatcaaagtatcacctttcatttgaagattgttcaaacggtcttcaaaaccagcaatttcttccatcattgccttgtggtgggccaattgctgggtgattgtctccaggctgcttgtctccaggaggtcaggtgccaccagtctgccagacatctgcagcagccacttttcgacctcttggagctcactgttgtagtcttcatggtctttgactttcgcctccagactgaagacatgctcctttcctatgctgcacaggtcctggtaatcactttgaagttgatctattttgtcctttaaagtgacgtcctgcaccagttccaaaagagcttcacccttctctctcactgactttactgatggttcatgggacagcaccgtttgttgaagtgacttgtatttagataactgagcttttttctcatataattccattttgggttcttcaggaacatgtagaatttcctggtattctgctatccactgtgtcagtgctttgcatttatctgagaattcctttgctaaatgaagacctttttccagcgtcatgtgttctttccggacagtgctggtcagttccttcaactgctccatgtgatcatgaatctcctttcttaacctctctgcctcgccttcctccaagtatttaacagccctctctcctttctcccgggctgatttcagcaaactgtgacctttctccatgtctttgagcaaaacctccaacgtcttcaatttcttccccatcattactgtatctactttgtcaatcttggtagccacattcttgaagtttttatgagtagagccataccaatcagaataggaactgagggatgattctgattcctccaaactctgaatctcctcctccaggaattttatttgttccagcacttggagaagcagggcctggtatctggaagtcagctgggtggcctggcaacccattctgctgttcacgtggctctcgtccagtatctcctgagctctagctcccacttcctcaacttcatctctgtatgcagtcacttcttcgtgccacttcttcatctgatgtaattgtatctccttggttgccctgttagactgacgtctggtcctgggactaactttctcctctgctgttttgagccattcatctacttgctgaaacttttgctccattagcctcaatttgttcaccacgttattgaactgagttcgagtctcggacagcctgtgctggtaagcctgccagtcttgccggagagactctaaagcccggtcctctgcctgtgggatacctgatgggatcacatcctctctggtgtgcagcactgagttcaacagggcctgcccctctgcacagtgtacctgtagctcctgaagatcacgcaatgttgtctcatgagtgtgggcatcaccttcaagaactgaatactggtcgagcttttcttgttcttgccccaaccaaacttcaaatgcctttaggtctctctgatactcttggtgcaggcggacaagtttttcagacttggttacggcttccttggccctctcttggatggctctgtatcgttcctgtagatcctggagttctagctgggtgacatagtgttctgtcatgccagcccctttgacttcgatggtctccagcaagctgctgtaactcagcacttcttcatttaataacttggcttttccgagcatcgttgttttatcccgcagctccgcatgctgcctttctgattcattcaggttggcttccatactatccatccaaccggagaactgtcgaacgccatcctgataacttgtccacttggagagagctccttcgagttggcttttacaacgaatccctgcagacaaaagggatgcccacatatccttcacactctgcagctgctgctgaatagtgggaatgccttctggagaagtattctgaaggacagattctcccctggtcactatcattttcatctgaatctctttttcctgtttgactgataatagagcctcgagcttgagcgtcctgctgtccagcacacttttgtcggatgtcgggtggcagtatgaatccagcatgtgaatcgcatccgtcatccagtcttgtaattctttaatcccaagagagaactgattgtgttctgcaacgattctatccagtcttgacactttctcctttgttaaattgcttagcgctagatactgagaagacagctgcgacactctgtgcctaaagctcttgctggcagcttgtccttcccacagctgctgagctttctctttcagcctgttgagctgaggctcgtagcagtgtatttcctcaaggacagactggagcttctgctgctccctcctctttgctggcagatcatagaggcgattgctgctttcatggaccatcttctcagttttactcagccagtcctggataggctcagcacttacttcaaagtccttcatttggatctttagattctctagagcagattctttttggtggagatttgaatgaaaatttttccaatcttcttttgcagctgtaactttggcctggatccctttcgctttctctttggtcagcagggtactcagaagttcccctttagacagcatcatgtttagcttgtgctgtccattttcactttctgacaaaaactcctgtattttctgaagactagttgaaacttcacttatattttgaggtatatcaaaacacttggcggtagtgatttttgcattaaccaaccactgctggaaatccctgaaggcctttcgaaatctttgctgtaaaatctgttctttattctggcagcccttggatgcttgcaaacaaagacaattatactctttaatcaagccagaaacttttccactgtaggtactcaggtctctggaaaatcgacaaagttcattcagctgagacttgagatcctctgttctaggctctgctttttgcaaagcatccagtatctcttgtcctttgtgccagcattccactatctcctcatccgtgttcttgccttccaggagggttaactgctgagcccaggttttcagaagggcactgaactgttccagggcctgctccagttgagccacttggcctgagaattcctgctccgaaagggccatctggctgaccaggttctccaaacagctctgcgtttggaatacactgtcttcccactgcttccagtcggcacgcagggcctgcatctccgtgtgcatgagctcacacccactggcagttgtgttctgtttcacttcgggagccagcgactccactctgctgagacggcttgcaccaatctctctggaatctatcagctccttaatttttgataactttttctgggtggctgatgaatctccagacatatctgaccaccggtgaagttcttcctttgctgaatggagccaatctgtgaactcgtggaccgcatctaaatacattagatgatctttcacaatctcttccactttcctcattttttccttggcaacagtcattatatcattaaactgtgttttcagctcctcttgagctgtgtccttgaaagactcatcctctgtcttttcgtagagctccctggacttcgcaattagacggtgaagggctctcgtgtgatcttctgcctcagacaggatggactggaggtggtcaagcaggacgaacttctctttcagacctggctgtggttgtaagggatgttctattttttgatccactgattccatccactgctccaactggtttttcctctctacatagtcattccattggctaatcacagactctaaagtgctttgagcgtggacggaggagctcatgatgtcagcccacacttctttaagggtctctaactgagtctgaatcaccctctgaccttctttgttgctacttctcaaggcctgttcccccttgccaatggccatattcaacttaacttccccttcacctttcatcaggagaatatcctgtatttgtgacagccgtttctccagggtgtctttgctcccaagagtgctctctgcacaggccagtctgtcctgaatggccttcacccagaaccacatgctttgcagtgcttcctccagggcttcgtgctcctgaagggccacctggcagctccggagtttctctttggtcattctaagtaggttctggtggcttgtgaggagctgggaacacaggcggccctcctgcccagcaccgtggccttcttcactcagaagctgccctctctgggaaagcttatcaagagactctcttgcagccagcagttctcccaaaaacatttcaactttatgaacttcatttttcttctcaggaatgtgctgtttactctctcccaagttttccgtattgaacctttcttccatttcatggatccataagttcagttttctgtgctgatcttcaaagcttccaagttctgaagcacagtcttgaagagcctgcttatctttaaggcattgtttcagaaatgcttgaaactcttcattggcctttgtgatttgttcttgaatgctactgacaatttgtttagacaaatgtgcatacaaagtttgtccttcttgagtcactgcatcaagtttgctctgcccatcactgactgagtccaaaatgttctgaagatcatggagctttgcttctagaactttgctgtcaccggtgcgatctgatgattcttttgctgctgcctttgctcccaaaaaccattcttggaattcctgcatagactcactgaagtgtttttccagagattcctgcaggctggcctgggttttggagcacaactggctcacggcttcatgtttctttatcagaccagtcattgcacggcccaggctctccaactcagctgagtggtacttgcggcacaagctattgagattttcttgggtagagctgatgttgctttgttgactttgaagttctttttgtatatccttgacttttttcaatgcttcacaagtctcattttgggcacagttcatcaacgattcttccacttttgtgaaccatgttgttatgtcattaataaacttctccacttgtgtactttgagccgtgaaatccttcagggttccttttgctacttcagttatttctttggcatgctccagtttctgcattaagtctgcttctataaactgaaggtctggcggtgtttctagatttttagttaattctttcagatcattaactttggaatgcagttcttccaatctcaatgctttgtttttaacttcagactcaaattctttaagcagttcttcagctctgaggtggttatccaggttgctgatgttttctgccatctgtggaacgcagttgtttgaccatccctcaatctcatctctagttgacagtacatcatcccaaatggacaggcttactctcagcctatccatgttttcttcaagtttctctgatacatccagccatttgtccacggtgctctccatgtctgttttcaccaagctgaaatcactactgtgaattttcttcagctcagataacaagtgttttcctttgctggtaaagttatccaagtctttctgtttgtaattcattttgttcttggcagtttcatgcttggaaaaagcccatttaagatcctcctgatcttttatggtagttctggttacaatcacactgctggcattttctaagactttagatacagctgatttcaggttctgatattctctcattaagtcaataagtccacagcactgaccctgattttcatgaattagtcttttggtatcatcccaggtgacctctaagcggtttatctccctgtcaacttcaggtgcaaaagctacatctttctgggcaatttgcttggctttgtctttcaaccaacatagttcatgctcgtgagaattcaattcatcttctagctgattaaacactcttaacctctgctgaagagcttggcgggtaggttctttcaatcgctctttgtcagtcctttcttcaatgtcctcaatgcttttcagaagctcctctttctggtcttggaatgcttttttcaacactgccagagcatctgcctcactctgcttggttcccagaaggttctggatcctctctacctctccacagagctgatcagccgtggctctgcaggaagtcctttgctcagagctcccgattttcagatggtattgggctttggaaagaatgccatccagactgacggcagcagattctaatgctttagcattttgaagagcatcattgaggtccttttctatcaaatcagactcgttcttattcatactgttggttgcttccactgtttgcctcagctggcggagaatgccggacagagaggcatggctctggaggaattctgccaaatgggacagggcaagctgccgcctctccacaacctggctggcctcctcaaacagctggaagcagtcctcagcctttccctgcaggaggtggaggtcctcagcacggcccagagaacccaactttgctaagtgaccctgcagactctgcaattcgccctttttgctctctacttctgctgcgtggtccttatgccgagtaagggctacttgatggtccattatgctaatctcagaggtagtttgtaattcactgagaaacagtttaatccagacagaaaaggaaagcagcagctcatcaaattgctggtgttcagcaaccacagactgaagaaaattaatccttttgttaatgatctgtggtaaatctctccatctctcatccaactgctccaaatgtagtttcatcattttcacatcatctttggaggctactgagaacaatgattccttcaattgcaaaagtttgctatagaatgaggcctgggatacaacttcattttgcagtgcctgtattaactgaagttcaccttccactttgactctgtctgcagaaatgtccatttctggggaactggctttagcttcaccccgctctaaccaggtcaaaaaggatgatagttctttctctagcctctgccagtgggccagcagattctccagcgccgtctgtctctccttcgccctccttaggatgtcctcgtattgctgctgtagagccgcagcctcctgaacacaggaatctctgttcacaaccttcctggcactggctgagaaggcagtgatcgcgctgctcagtgactccagggcctggcagagatccatatgttcttgaagaactttgtatgtttctgtagctgaagaacatattttaattggaacagcaagtttatcttcaaattcagacacagattgctggatctttctaaggttctcttcaaacttttgctgctgagataaatgtcccaggattgttccttccagacactgtgcatgctctcgaagctcttccccgtatcttcttatttgtgtcaacttggctttaattcgagcagattctccagtggtaacaaactgagcaaaagactgggcttcttcttctaatcctacaatgctgctgagcttactttctatttcctgaattgtgaccttaatttggctgatttgcatgtccatggcagatgacgaagtttccaaggcattgagttctttttctttctcagttatccagacggacagagtctcaaaattactgccaaaatgatcccacttggttttcaccatttccatggttttaatatcttcttcaagcgtgtcttctaattttttgacttgttctttgattgacttggcctgctgttgaagcagctgcttattttggggcccaagcggtatctctgaagcttcctttacaaggttctcagcctggactgcaatactttctgtccgtttagaaaactcctttgtttgttccagttctgaagataaactttccaaactgctaaaactcaagaagcgttcatgactggaacctgtttgaaaaaggtatcttactactgtttctttgtttgtttcaaatcgctcccattttcttaatgtgacctggatgcggcgttcctgcctctcccggctgcgctccaggccatccagtgtgctctccagcttccgcagctcctcgtggcctcggtcaggcagccccccttctccctgctgcgcctgcgcgatctgctgctgcacatctctcttctttgctgagatccgctttgtcttttgctggtgatgaagaagtaactgctgtgcttcaaacagattttcagtatccaagatcttctcagcttgttcctggacttctttagagccagaaattaattcttcgagagaatttttgactatttctttgtactggacacagtccccaaaattgcttagcatcttttcaacctctgacagcagcgtcacaagagccttgaaagagctggataattttgccagctcatctccctgcttttgggcttcattctcagaagaaacttctgtcaaaactttcagcctggatttcagccagctgagggtctcaccccttttggtaacaccatttctgatctcttcaacggcacgtttaacctctccgtggttggcagtatcgatggcctcacccttgatcccctttaattgtgtctcatttgtagatatccaagatgagaactcagagaatctgctagtgtagtccttccacttgtctgggtcttccatgagcttcctgtaggtgctgtcaatggcagctctgagctctttgagagtcacgtgacaggttccaggtgtgtcccttactgggtcccgcactgggagtttcacacagagttcctcgatgagctgtaaccttttctcacagagatgatgaggacctttgtcactgaagaaaaccctgtgctctttaattatcttttcactgccttcctggggcatcagcttggtctctcgatccagctcagttctgcattcttctacagaggctaagaacctattcttctccacatcaatcttcagatgaagcaaatgataaggggcttctccttgaagatccttccattgtttgtggagctttcgaacagcttcctgcagcccctgctgctcctgctctggaaggatgtcggtgagttcatcacaagctttcaggaaagcattgagcaccctctgatccagctgactgaaaaactcagtgtgtctccgcaggagctcctctggatcccccttttcctccaggccctcctgagcaatccgcagtaccttctccaactctgctcgagactcctcaaacttcttcatcaagcgactgttggtttccacatgcttcttccaatctccagttttctttaccatactctgaaaagcaacatgaatatctgcaatctgtctttgtagcctcgtctgatcaaaatgctttaacacgttgctcaaggtcacaaacttttgaacactttgactgcctttctcaataagtgtcaaggttttcttacagttttcttgacaagctaacagttcctgatgtttttgtttaaaaagggcactcgattgtgcctcacgctcaagaactgtgataatttcattgattttcccaagtgagtcataaaaggacgtcatctgcttttctaattcctccaacggaatcaacagctgctgagactcataaaggagtggggagtaacattctttgaccttggttagctgctctttgagctttgacatggtcgcaaacatttcttttccttcttcttgggggctttctttggtaatgaggtgtgctgtctttgtaattatcttgtattgggcatccatcacaggcaccctctgctcaatatcctccaagtcttgaattaatagcttgacattcataaaagagacttctaagggttcagaaagtttcttatgggcttccgttgcaaaagcagacagggtaacaacacagtctgtgtattccttcttcattctgtccatctcatcagcttgagcatattgcttgacttccataaacaactccctccaccgcccatttagcaacagtaattgctgcttcaggtcacgggaaaccatctcatcacaggtttcaattagaaaattgccagcatcgttcatggcagtatgctgctgaatccaatgaggtaaatttcgaaaaaaatcctttttggcattttctgattgattgagcattttttcagcatcctctagccaggcttgcagactagccactgtattgccatagcgatcccagttagagatcacttcttccagcatgctcctcacactcctcacttctactgagagattcctccactgagcggtggtttcattcatgaatttcatcacattctcagcttcttccactgaaccatctgctttgacatacatctcagctgtctgtttcaagatctggtatgtcacctcatattgttcaaagaacttgctattttctataaaagacacgtagttttgtagaagctgctccactgactctctcctcccgtacttaatgatccaagacttcagctttgactctgcaagaaccagcagtgagagcagacggtactttaattctaaaaattccattttcattaggtgtagctctgatgtggaggaaacaaaatgaaacctctcggccatgtcctctaattgatcaggtggcactggaatcccgttaacagacctggtccggtagatttcatggaatgctcttttgtgggcatccgtgttttgaagcagatccttatgttgctcaagtttccgttgtatcgtgtttgctgtttcctcgtggacctgttgaacggttatttcctctctcagggccacctccgctctgtacagccaggcacctatggtgcccagaggtgcaggaagagatttatcaagctgtatatgccagtcaaagagcctggaggtcactctatcccaagattgttttaccaatgcttggtcaagtgacaatttaccgtctctgtgtaatggttgtattaaatgttcaatctgtttcctcttcatttcatattgaactctgaagtgcttaaatgactgatatttatcctgtaaatttgattccaccatctgtgctcttgtcaaatctctctcaaattgttctatccaaactttcatttccttaaaaattactctgtcttctctcttaaaattttgtacagaatttgcaaaagatgggaaacctggaagtatttcatcatcctcttgcccatcagtgcttgcattgtggatgtcaggataatgtttcagaaactgggctacataggtcataatagatttctcatctggtttatccacatcaacgtcttcaggatctagcagtcttgggatccccagttctgtttcggcgatagtgaaagcatcctccaaattttctcggttggatctgcctttcactgtctccaagtccaccaattccggtcgaatggcatgaataactgaatgaaaggcaaccccgcttctccaactcttcccaaaatcttttacttctattccagtctgcttgccagctgtgtactgaacccactttaataaagccttcttagcatttccttggatcttggtggtcaccttccgtttacttggtgggctgggagtctcagagctaactatgctgtccacggaggatgcgctgctggacaaagactggagctggggcaggttgctggtcaactcttcaatctggaaatatagaataatggtccacatcaatccaagaactattgagggtcggccatcagctatatcggtggagttaatgttgactaatttaatctttcttccttcgaggaacttgagtgccgtgccaatgttagccacagcatggattcgcttcatccggcgtccttgttcacaaggcagtttctgcccagacaggacctccagaagggcaagcagtttaacaccatctttcatgtcttcaaaaagatcgtccaccaccattggaggtttccgcttggccagatgagagttgatccattttgtgaaagttcgtttttgtactatctcttgctcatcttgcagcctctgcatcacattggcgatatcccgaggacaccgggaggcccctctggaggttgccatggtccctccggaagcacgaagccaacaccaagagactcttcactggaggcagcacagggctacaccactctagaaaacatgcttggacttttctagatctattctgtcataaatgaattccaggcctttgcagcactcaacaaggaggcagctctcccaaagactgaactgcttctttttcttcttccgttttaagactgtcctcttacatgaactcaagaaccttctctctcggcctcgttcagtttcccagcagcaaggcgaagcgagcgaacgcttcctcccggctctctgcgcccaggctcggcgggaccccggggatgcgcggctgtccgcccgccctgtcgccgggatcgggcgcggtctgcaggactgcgggagcccagccgccctcctggagatgcacggccttgggcgtttctccgcagctgcaaagctgtgctgtgacccacccgctcagcgagcctttataccgggaccacctcccgggggtcgaggtgggaaggaaatgtccctgagagccgggacgcgctgcctccgctgcctggaggagctgcgctgtcct

SEQ ID NO: 9577 - RNA, 14216 nt, Homo sapiens
  source 1..14216: mol_type = other RNA
agttcttcagtggcaagctttatcaaaatcttccttaaaatgcttcctagaaaccaaattcttctctagttcttgtaaccggtgactgcacttttgtaaaacactgtcatagacactctgcaattcctgaagcttccccagcacttcactcttttcctgctctgtgacttccttcattagttcgcgaccctgggcccaaagtccagtgacttcattttggtaagtcttgaggctggcttgtgcactcttacatgttttgacttgtttgctcacatcatctggtaacagacagatgtgttcacggaacattatctttcgctcatgttgctgaatttggctggtggcctggaacactgccatgagaaactgggttttctcggacaaggctttgtttaagtactttcttcgctggcccactaagtcactgagacaattcacgtggctttgtgcatcagagagagccttctggatgacctgtcgctcattgagaccaagatctgccatgaccctgtctgcgtcctttataagcgatttcaggagcatctgcttggcctccagttcactgcagatggccaggtgatccatgagaaggttctgagccatatctggaggagggctctgcttaagggcctcggcgatgttgggttgttgctcttctgcccactccattagctcctgaaatctggactgcaccacatttaactcctccaagttggtgactgacacttggattttccttttaatgaggtcctcaagctgaaaccaacgttgctctaaatgactcgtctgttctttgactaactccttgtcatctaaattcagatgctctatcattttctgcttttgatctttcagatcttcaatagcatactttctctcctgcaatgccaatgctaactttttcaaagcttccaggtggacagctgtactctctgcatcagatctggccaagttatcccattctgtagtaaatttttctaggaacacttcaacaacattcatacagtcatggtaatctcttgttctctgaagatcctcttccctttgcaagcacaggttgttagactgacggcacaaatcgagccactgatcatttaaatgatttatttccttgtgttcaggcgattcctccttctttgttaacttattcaccttttctattatggtgttcacggatgcctgtttgctctgtagtttcttaacaaaatccttaacttgtgaaaccatgttctgtgcaatgttcagctccagctcagagtgcctcctcttcatgttctgcagttgctgatcagcatcttgcaggtaaatccagagctcagacttcaggtgcttgatctcttcccagccctgagttaagttctgggcctggacaagcttttgttcaatcgtttgctctgtttgttgaatgtcttttgctgtggttttcaccgaagcatttgacaggtcacacatggagcaaaggagatctaggtaggtccttgcctgctcttgcaaagctctgaagtgtttgacctgcttaatggcttctgccctactaagaggtggttgaggacttggctctaaatccggctggactgcagaaagccaggcctggcactgctgcagggtgtcttgtcggctgacgtgcttctgaagttcgtgttccaaactctggtacatcctctgagctgtgctgcagatcgctgagtagctgtcctttgtgccctgcagatgagcatgcacgttttgtttaagtttcgcttgcaggtggtctgcacattggccaatcaaagtatcacctttcatttgaagattgttcaaacggtcttcaaaaccagcaatttcttccatcattgccttgtggtgggccaattgctgggtgattgtctccaggctgcttgtctccaggaggtcaggtgccaccagtctgccagacatctgcagcagccacttttcgacctcttggagctcactgttgtagtcttcatggtctttgactttcgcctccagactgaagacatgctcctttcctatgctgcacaggtcctggtaatcactttgaagttgatctattttgtcctttaaagtgacgtcctgcaccagttccaaaagagcttcacccttctctctcactgactttactgatggttcatgggacagcaccgtttgttgaagtgacttgtatttagataactgagcttttttctcatataattccattttgggttcttcaggaacatgtagaatttcctggtattctgctatccactgtgtcagtgctttgcatttatctgagaattcctttgctaaatgaagacctttttccagcgtcatgtgttctttccggacagtgctggtcagttccttcaactgctccatgtgatcatgaatctcctttcttaacctctctgcctcgccttcctccaagtatttaacagccctctctcctttctcccgggctgatttcagcaaactgtgacctttctccatgtctttgagcaaaacctccaacgtcttcaatttcttccccatcattactgtatctactttgtcaatcttggtagccacattcttgaagtttttatgagtagagccataccaatcagaataggaactgagggatgattctgattcctccaaactctgaatctcctcctccaggaattttatttgttccagcacttggagaagcagggcctggtatctggaagtcagctgggtggcctggcaacccattctgctgttcacgtggctctcgtccagtatctcctgagctctagctcccacttcctcaacttcatctctgtatgcagtcacttcttcgtgccacttcttcatctgatgtaattgtatctccttggttgccctgttagactgacgtctggtcctgggactaactttctcctctgctgttttgagccattcatctacttgctgaaacttttgctccattagcctcaatttgttcaccacgttattgaactgagttcgagtctcggacagcctgtgctggtaagcctgccagtcttgccggagagactctaaagcccggtcctctgcctgtgggatacctgatgggatcacatcctctctggtgtgcagcactgagttcaacagggcctgcccctctgcacagtgtacctgtagctcctgaagatcacgcaatgttgtctcatgagtgtgggcatcaccttcaagaactgaatactggtcgagcttttcttgttcttgccccaaccaaacttcaaatgcctttaggtctctctgatactcttggtgcaggcggacaagtttttcagacttggttacggcttccttggccctctcttggatggctctgtatcgttcctgtagatcctggagttctagctgggtgacatagtgttctgtcatgccagcccctttgacttcgatggtctccagcaagctgctgtaactcagcacttcttcatttaataacttggcttttccgagcatcgttgttttatcccgcagctccgcatgctgcctttctgattcattcaggttggcttccatactatccatccaaccggagaactgtcgaacgccatcctgataacttgtccacttggagagagctccttcgagttggcttttacaacgaatccctgcagacaaaagggatgcccacatatccttcacactctgcagctgctgctgaatagtgggaatgccttctggagaagtattctgaaggacagattctcccctggtcactatcattttcatctgaatctctttttcctgtttgactgataatagagcctcgagcttgagcgtcctgctgtccagcacacttttgtcggatgtcgggtggcagtatgaatccagcatgtgaatcgcatccgtcatccagtcttgtaattctttaatcccaagagagaactgattgtgttctgcaacgattctatccagtcttgacactttctcctttgttaaattgcttagcgctagatactgagaagacagctgcgacactctgtgcctaaagctcttgctggcagcttgtccttcccacagctgctgagctttctctttcagcctgttgagctgaggctcgtagcagtgtatttcctcaaggacagactggagcttctgctgctccctcctctttgctggcagatcatagaggcgattgctgctttcatggaccatcttctcagttttactcagccagtcctggataggctcagcacttacttcaaagtccttcatttggatctttagattctctagagcagattctttttggtggagatttgaatgaaaatttttccaatcttcttttgcagctgtaactttggcctggatccctttcgctttctctttggtcagcagggtactcagaagttcccctttagacagcatcatgtttagcttgtgctgtccattttcactttctgacaaaaactcctgtattttctgaagactagttgaaacttcacttatattttgaggtatatcaaaacacttggcggtagtgatttttgcattaaccaaccactgctggaaatccctgaaggcctttcgaaatctttgctgtaaaatctgttctttattctggcagcccttggatgcttgcaaacaaagacaattatactctttaatcaagccagaaacttttccactgtaggtactcaggtctctggaaaatcgacaaagttcattcagctgagacttgagatcctctgttctaggctctgctttttgcaaagcatccagtatctcttgtcctttgtgccagcattccactatctcctcatccgtgttcttgccttccaggagggttaactgctgagcccaggttttcagaagggcactgaactgttccagggcctgctccagttgagccacttggcctgagaattcctgctccgaaagggccatctggctgaccaggttctccaaacagctctgcgtttggaatacactgtcttcccactgcttccagtcggcacgcagggcctgcatctccgtgtgcatgagctcacacccactggcagttgtgttctgtttcacttcgggagccagcgactccactctgctgagacggcttgcaccaatctctctggaatctatcagctccttaatttttgataactttttctgggtggctgatgaatctccagacatatctgaccaccggtgaagttcttcctttgctgaatggagccaatctgtgaactcgtggaccgcatctaaatacattagatgatctttcacaatctcttccactttcctcattttttccttggcaacagtcattatatcattaaactgtgttttcagctcctcttgagctgtgtccttgaaagactcatcctctgtcttttcgtagagctccctggacttcgcaattagacggtgaagggctctcgtgtgatcttctgcctcagacaggatggactggaggtggtcaagcaggacgaacttctctttcagacctggctgtggttgtaagggatgttctattttttgatccactgattccatccactgctccaactggtttttcctctctacatagtcattccattggctaatcacagactctaaagtgctttgagcgtggacggaggagctcatgatgtcagcccacacttctttaagggtctctaactgagtctgaatcaccctctgaccttctttgttgctacttctcaaggcctgttcccccttgccaatggccatattcaacttaacttccccttcacctttcatcaggagaatatcctgtatttgtgacagccgtttctccagggtgtctttgctcccaagagtgctctctgcacaggccagtctgtcctgaatggccttcacccagaaccacatgctttgcagtgcttcctccagggcttcgtgctcctgaagggccacctggcagctccggagtttctctttggtcattctaagtaggttctggtggcttgtgaggagctgggaacacaggcggccctcctgcccagcaccgtggccttcttcactcagaagctgccctctctgggaaagcttatcaagagactctcttgcagccagcagttctcccaaaaacatttcaactttatgaacttcatttttcttctcaggaatgtgctgtttactctctcccaagttttccgtattgaacctttcttccatttcatggatccataagttcagttttctgtgctgatcttcaaagcttccaagttctgaagcacagtcttgaagagcctgcttatctttaaggcattgtttcagaaatgcttgaaactcttcattggcctttgtgatttgttcttgaatgctactgacaatttgtttagacaaatgtgcatacaaagtttgtccttcttgagtcactgcatcaagtttgctctgcccatcactgactgagtccaaaatgttctgaagatcatggagctttgcttctagaactttgctgtcaccggtgcgatctgatgattcttttgctgctgcctttgctcccaaaaaccattcttggaattcctgcatagactcactgaagtgtttttccagagattcctgcaggctggcctgggttttggagcacaactggctcacggcttcatgtttctttatcagaccagtcattgcacggcccaggctctccaactcagctgagtggtacttgcggcacaagctattgagattttcttgggtagagctgatgttgctttgttgactttgaagttctttttgtatatccttgacttttttcaatgcttcacaagtctcattttgggcacagttcatcaacgattcttccacttttgtgaaccatgttgttatgtcattaataaacttctccacttgtgtactttgagccgtgaaatccttcagggttccttttgctacttcagttatttctttggcatgctccagtttctgcattaagtctgcttctataaactgaaggtctggcggtgtttctagatttttagttaattctttcagatcattaactttggaatgcagttcttccaatctcaatgctttgtttttaacttcagactcaaattctttaagcagttcttcagctctgaggtggttatccaggttgctgatgttttctgccatctgtggaacgcagttgtttgaccatccctcaatctcatctctagttgacagtacatcatcccaaatggacaggcttactctcagcctatccatgttttcttcaagtttctctgatacatccagccatttgtccacggtgctctccatgtctgttttcaccaagctgaaatcactactgtgaattttcttcagctcagataacaagtgttttcctttgctggtaaagttatccaagtctttctgtttgtaattcattttgttcttggcagtttcatgcttggaaaaagcccatttaagatcctcctgatcttttatggtagttctggttacaatcacactgctggcattttctaagactttagatacagctgatttcaggttctgatattctctcattaagtcaataagtccacagcactgaccctgattttcatgaattagtcttttggtatcatcccaggtgacctctaagcggtttatctccctgtcaacttcaggtgcaaaagctacatctttctgggcaatttgcttggctttgtctttcaaccaacatagttcatgctcgtgagaattcaattcatcttctagctgattaaacactcttaacctctgctgaagagcttggcgggtaggttctttcaatcgctctttgtcagtcctttcttcaatgtcctcaatgcttttcagaagctcctctttctggtcttggaatgcttttttcaacactgccagagcatctgcctcactctgcttggttcccagaaggttctggatcctctctacctctccacagagctgatcagccgtggctctgcaggaagtcctttgctcagagctcccgattttcagatggtattgggctttggaaagaatgccatccagactgacggcagcagattctaatgctttagcattttgaagagcatcattgaggtccttttctatcaaatcagactcgttcttattcatactgttggttgcttccactgtttgcctcagctggcggagaatgccggacagagaggcatggctctggaggaattctgccaaatgggacagggcaagctgccgcctctccacaacctggctggcctcctcaaacagctggaagcagtcctcagcctttccctgcaggaggtggaggtcctcagcacggcccagagaacccaactttgctaagtgaccctgcagactctgcaattcgccctttttgctctctacttctgctgcgtggtccttatgccgagtaagggctacttgatggtccattatgctaatctcagaggtagtttgtaattcactgagaaacagtttaatccagacagaaaaggaaagcagcagctcatcaaattgctggtgttcagcaaccacagactgaagaaaattaatccttttgttaatgatctgtggtaaatctctccatctctcatccaactgctccaaatgtagtttcatcattttcacatcatctttggaggctactgagaacaatgattccttcaattgcaaaagtttgctatagaatgaggcctgggatacaacttcattttgcagtgcctgtattaactgaagttcaccttccactttgactctgtctgcagaaatgtccatttctggggaactggctttagcttcaccccgctctaaccaggtcaaaaaggatgatagttctttctctagcctctgccagtgggccagcagattctccagcgccgtctgtctctccttcgccctccttaggatgtcctcgtattgctgctgtagagccgcagcctcctgaacacaggaatctctgttcacaaccttcctggcactggctgagaaggcagtgatcgcgctgctcagtgactccagggcctggcagagatccatatgttcttgaagaactttgtatgtttctgtagctgaagaacatattttaattggaacagcaagtttatcttcaaattcagacacagattgctggatctttctaaggttctcttcaaacttttgctgctgagataaatgtcccaggattgttccttccagacactgtgcatgctctcgaagctcttccccgtatcttcttatttgtgtcaacttggctttaattcgagcagattctccagtggtaacaaactgagcaaaagactgggcttcttcttctaatcctacaatgctgctgagcttactttctatttcctgaattgtgaccttaatttggctgatttgcatgtccatggcagatgacgaagtttccaaggcattgagttctttttctttctcagttatccagacggacagagtctcaaaattactgccaaaatgatcccacttggttttcaccatttccatggttttaatatcttcttcaagcgtgtcttctaattttttgacttgttctttgattgacttggcctgctgttgaagcagctgcttattttggggcccaagcggtatctctgaagcttcctttacaaggttctcagcctggactgcaatactttctgtccgtttagaaaactcctttgtttgttccagttctgaagataaactttccaaactgctaaaactcaagaagcgttcatgactggaacctgtttgaaaaaggtatcttactactgtttctttgtttgtttcaaatcgctcccattttcttaatgtgacctggatgcggcgttcctgcctctcccggctgcgctccaggccatccagtgtgctctccagcttccgcagctcctcgtggcctcggtcaggcagccccccttctccctgctgcgcctgcgcgatctgctgctgcacatctctcttctttgctgagatccgctttgtcttttgctggtgatgaagaagtaactgctgtgcttcaaacagattttcagtatccaagatcttctcagcttgttcctggacttctttagagccagaaattaattcttcgagagaatttttgactatttctttgtactggacacagtccccaaaattgcttagcatcttttcaacctctgacagcagcgtcacaagagccttgaaagagctggataattttgccagctcatctccctgcttttgggcttcattctcagaagaaacttctgtcaaaactttcagcctggatttcagccagctgagggtctcaccccttttggtaacaccatttctgatctcttcaacggcacgtttaacctctccgtggttggcagtatcgatggcctcacccttgatcccctttaattgtgtctcatttgtagatatccaagatgagaactcagagaatctgctagtgtagtccttccacttgtctgggtcttccatgagcttcctgtaggtgctgtcaatggcagctctgagctctttgagagtcacgtgacaggttccaggtgtgtcccttactgggtcccgcactgggagtttcacacagagttcctcgatgagctgtaaccttttctcacagagatgatgaggacctttgtcactgaagaaaaccctgtgctctttaattatcttttcactgccttcctggggcatcagcttggtctctcgatccagctcagttctgcattcttctacagaggctaagaacctattcttctccacatcaatcttcagatgaagcaaatgataaggggcttctccttgaagatccttccattgtttgtggagctttcgaacagcttcctgcagcccctgctgctcctgctctggaaggatgtcggtgagttcatcacaagctttcaggaaagcattgagcaccctctgatccagctgactgaaaaactcagtgtgtctccgcaggagctcctctggatcccccttttcctccaggccctcctgagcaatccgcagtaccttctccaactctgctcgagactcctcaaacttcttcatcaagcgactgttggtttccacatgcttcttccaatctccagttttctttaccatactctgaaaagcaacatgaatatctgcaatctgtctttgtagcctcgtctgatcaaaatgctttaacacgttgctcaaggtcacaaacttttgaacactttgactgcctttctcaataagtgtcaaggttttcttacagttttcttgacaagctaacagttcctgatgtttttgtttaaaaagggcactcgattgtgcctcacgctcaagaactgtgataatttcattgattttcccaagtgagtcataaaaggacgtcatctgcttttctaattcctccaacggaatcaacagctgctgagactcataaaggagtggggagtaacattctttgaccttggttagctgctctttgagctttgacatggtcgcaaacatttcttttccttcttcttgggggctttctttggtaatgaggtgtgctgtctttgtaattatcttgtattgggcatccatcacaggcaccctctgctcaatatcctccaagtcttgaattaatagcttgacattcataaaagagacttctaagggttcagaaagtttcttatgggcttccgttgcaaaagcagacagggtaacaacacagtctgtgtattccttcttcattctgtccatctcatcagcttgagcatattgcttgacttccataaacaactccctccaccgcccatttagcaacagtaattgctgcttcaggtcacgggaaaccatctcatcacaggtttcaattagaaaattgccagcatcgttcatggcagtatgctgctgaatccaatgaggtaaatttcgaaaaaaatcctttttggcattttctgattgattgagcattttttcagcatcctctagccaggcttgcagactagccactgtattgccatagcgatcccagttagagatcacttcttccagcatgctcctcacactcctcacttctactgagagattcctccactgagcggtggtttcattcatgaatttcatcacattctcagcttcttccactgaaccatctgctttgacatacatctcagctgtctgtttcaagatctggtatgtcacctcatattgttcaaagaacttgctattttctataaaagacacgtagttttgtagaagctgctccactgactctctcctcccgtacttaatgatccaagacttcagctttgactctgcaagaaccagcagtgagagcagacggtactttaattctaaaaattccattttcattaggtgtagctctgatgtggaggaaacaaaatgaaacctctcggccatgtcctctaattgatcaggtggcactggaatcccgttaacagacctggtccggtagatttcatggaatgctcttttgtgggcatccgtgttttgaagcagatccttatgttgctcaagtttccgttgtatcgtgtttgctgtttcctcgtggacctgttgaacggttatttcctctctcagggccacctccgctctgtacagccaggcacctatggtgcccagaggtgcaggaagagatttatcaagctgtatatgccagtcaaagagcctggaggtcactctatcccaagattgttttaccaatgcttggtcaagtgacaatttaccgtctctgtgtaatggttgtattaaatgttcaatctgtttcctcttcatttcatattgaactctgaagtgcttaaatgactgatatttatcctgtaaatttgattccaccatctgtgctcttgtcaaatctctctcaaattgttctatccaaactttcatttccttaaaaattactctgtcttctctcttaaaattttgtacagaatttgcaaaagatgggaaacctggaagtatttcatcatcctcttgcccatcagtgcttgcattgtggatgtcaggataatgtttcagaaactgggctacataggtcataatagatttctcatctggtttatccacatcaacgtcttcaggatctagcagtcttgggatccccagttctgtttcggcgatagtgaaagcatcctccaaattttctcggttggatctgcctttcactgtctccaagtccaccaattccggtcgaatggcatgaataactgaatgaaaggcaaccccgcttctccaactcttcccaaaatcttttacttctattccagtctgcttgccagctgtgtactgaacccactttaataaagccttcttagcatttccttggatcttggtggtcaccttccgtttacttggtgggctgggagtctcagagctaactatgctgtccacggaggatgcgctgctggacaaagactggagctggggcaggttgctggtcaactcttcaatctggaaatatagaataatggtccacatcaatccaagaactattgagggtcggccatcagctatatcggtggagttaatgttgactaatttaatctttcttccttcgaggaacttgagtgccgtgccaatgttagccacagcatggattcgcttcatccggcgtccttgttcacaaggcagtttctgcccagacaggacctccagaagggcaagcagtttaacaccatctttcatgtcttcaaaaagatcgtccaccaccattggaggtttccgcttggccagatgagagttgatccattttgtgaaagttcgtttttgtactatctcttgctcatcttgcagcctctgcatcacattggcgatatcccgaggacaccgggaggcccctctggaggttgccatggtccctccggaagcacgaagccaacaccaagagactcttcactggaggcagcacagggctacaccactctagaaaacatgcttggacttttctagatctattctgtcataaatgaattccaggcctttgcagcactcaacaaggaggcagctctcccaaagactgaactgcttctttttcttcttccgttttaagactgtcctcttacatgaactcaagaaccttctctctcggcctcgttcagtttcccagcagcaaggcgaagcgagcgaacgcttcctcccggctctctgcgcccaggctcggcgggaccccggggatgcgcggctgtccgcccgccctgtcgccgggatcgggcgcggtctgcaggactgcgggagcccagccgccctggtgacagaggacaacaatctcagcccgctgcggccggcggccgcggcccggcgcccgcgctcaccctggctggctcgcccacact

SEQ ID NO: 9578 - RNA, 12320 nt, Homo sapiens
  source 1..12320: mol_type = other RNA
agttcttcagtggcaagctttatcaaaatcttccttaaaatgcttcctagaaaccaaattcttctctagttcttgtaaccggtgactgcacttttgtaaaacactgtcatagacactctgcaattcctgaagcttccccagcacttcactcttttcctgctctgtgacttccttcattagttcgcgaccctgggcccaaagtccagtgacttcattttggtaagtcttgaggctggcttgtgcactcttacatgttttgacttgtttgctcacatcatctggtaacagacagatgtgttcacggaacattatctttcgctcatgttgctgaatttggctggtggcctggaacactgccatgagaaactgggttttctcggacaaggctttgtttaagtactttcttcgctggcccactaagtcactgagacaattcacgtggctttgtgcatcagagagagccttctggatgacctgtcgctcattgagaccaagatctgccatgaccctgtctgcgtcctttataagcgatttcaggagcatctgcttggcctccagttcactgcagatggccaggtgatccatgagaaggttctgagccatatctggaggagggctctgcttaagggcctcggcgatgttgggttgttgctcttctgcccactccattagctcctgaaatctggactgcaccacatttaactcctccaagttggtgactgacacttggattttccttttaatgaggtcctcaagctgaaaccaacgttgctctaaatgactcgtctgttctttgactaactccttgtcatctaaattcagatgctctatcattttctgcttttgatctttcagatcttcaatagcatactttctctcctgcaatgccaatgctaactttttcaaagcttccaggtggacagctgtactctctgcatcagatctggccaagttatcccattctgtagtaaatttttctaggaacacttcaacaacattcatacagtcatggtaatctcttgttctctgaagatcctcttccctttgcaagcacaggttgttagactgacggcacaaatcgagccactgatcatttaaatgatttatttccttgtgttcaggcgattcctccttctttgttaacttattcaccttttctattatggtgttcacggatgcctgtttgctctgtagtttcttaacaaaatccttaacttgtgaaaccatgttctgtgcaatgttcagctccagctcagagtgcctcctcttcatgttctgcagttgctgatcagcatcttgcaggtaaatccagagctcagacttcaggtgcttgatctcttcccagccctgagttaagttctgggcctggacaagcttttgttcaatcgtttgctctgtttgttgaatgtcttttgctgtggttttcaccgaagcatttgacaggtcacacatggagcaaaggagatctaggtaggtccttgcctgctcttgcaaagctctgaagtgtttgacctgcttaatggcttctgccctactaagaggtggttgaggacttggctctaaatccggctggactgcagaaagccaggcctggcactgctgcagggtgtcttgtcggctgacgtgcttctgaagttcgtgttccaaactctggtacatcctctgagctgtgctgcagatcgctgagtagctgtcctttgtgccctgcagatgagcatgcacgttttgtttaagtttcgcttgcaggtggtctgcacattggccaatcaaagtatcacctttcatttgaagattgttcaaacggtcttcaaaaccagcaatttcttccatcattgccttgtggtgggccaattgctgggtgattgtctccaggctgcttgtctccaggaggtcaggtgccaccagtctgccagacatctgcagcagccacttttcgacctcttggagctcactgttgtagtcttcatggtctttgactttcgcctccagactgaagacatgctcctttcctatgctgcacaggtcctggtaatcactttgaagttgatctattttgtcctttaaagtgacgtcctgcaccagttccaaaagagcttcacccttctctctcactgactttactgatggttcatgggacagcaccgtttgttgaagtgacttgtatttagataactgagcttttttctcatataattccattttgggttcttcaggaacatgtagaatttcctggtattctgctatccactgtgtcagtgctttgcatttatctgagaattcctttgctaaatgaagacctttttccagcgtcatgtgttctttccggacagtgctggtcagttccttcaactgctccatgtgatcatgaatctcctttcttaacctctctgcctcgccttcctccaagtatttaacagccctctctcctttctcccgggctgatttcagcaaactgtgacctttctccatgtctttgagcaaaacctccaacgtcttcaatttcttccccatcattactgtatctactttgtcaatcttggtagccacattcttgaagtttttatgagtagagccataccaatcagaataggaactgagggatgattctgattcctccaaactctgaatctcctcctccaggaattttatttgttccagcacttggagaagcagggcctggtatctggaagtcagctgggtggcctggcaacccattctgctgttcacgtggctctcgtccagtatctcctgagctctagctcccacttcctcaacttcatctctgtatgcagtcacttcttcgtgccacttcttcatctgatgtaattgtatctccttggttgccctgttagactgacgtctggtcctgggactaactttctcctctgctgttttgagccattcatctacttgctgaaacttttgctccattagcctcaatttgttcaccacgttattgaactgagttcgagtctcggacagcctgtgctggtaagcctgccagtcttgccggagagactctaaagcccggtcctctgcctgtgggatacctgatgggatcacatcctctctggtgtgcagcactgagttcaacagggcctgcccctctgcacagtgtacctgtagctcctgaagatcacgcaatgttgtctcatgagtgtgggcatcaccttcaagaactgaatactggtcgagcttttcttgttcttgccccaaccaaacttcaaatgcctttaggtctctctgatactcttggtgcaggcggacaagtttttcagacttggttacggcttccttggccctctcttggatggctctgtatcgttcctgtagatcctggagttctagctgggtgacatagtgttctgtcatgccagcccctttgacttcgatggtctccagcaagctgctgtaactcagcacttcttcatttaataacttggcttttccgagcatcgttgttttatcccgcagctccgcatgctgcctttctgattcattcaggttggcttccatactatccatccaaccggagaactgtcgaacgccatcctgataacttgtccacttggagagagctccttcgagttggcttttacaacgaatccctgcagacaaaagggatgcccacatatccttcacactctgcagctgctgctgaatagtgggaatgccttctggagaagtattctgaaggacagattctcccctggtcactatcattttcatctgaatctctttttcctgtttgactgataatagagcctcgagcttgagcgtcctgctgtccagcacacttttgtcggatgtcgggtggcagtatgaatccagcatgtgaatcgcatccgtcatccagtcttgtaattctttaatcccaagagagaactgattgtgttctgcaacgattctatccagtcttgacactttctcctttgttaaattgcttagcgctagatactgagaagacagctgcgacactctgtgcctaaagctcttgctggcagcttgtccttcccacagctgctgagctttctctttcagcctgttgagctgaggctcgtagcagtgtatttcctcaaggacagactggagcttctgctgctccctcctctttgctggcagatcatagaggcgattgctgctttcatggaccatcttctcagttttactcagccagtcctggataggctcagcacttacttcaaagtccttcatttggatctttagattctctagagcagattctttttggtggagatttgaatgaaaatttttccaatcttcttttgcagctgtaactttggcctggatccctttcgctttctctttggtcagcagggtactcagaagttcccctttagacagcatcatgtttagcttgtgctgtccattttcactttctgacaaaaactcctgtattttctgaagactagttgaaacttcacttatattttgaggtatatcaaaacacttggcggtagtgatttttgcattaaccaaccactgctggaaatccctgaaggcctttcgaaatctttgctgtaaaatctgttctttattctggcagcccttggatgcttgcaaacaaagacaattatactctttaatcaagccagaaacttttccactgtaggtactcaggtctctggaaaatcgacaaagttcattcagctgagacttgagatcctctgttctaggctctgctttttgcaaagcatccagtatctcttgtcctttgtgccagcattccactatctcctcatccgtgttcttgccttccaggagggttaactgctgagcccaggttttcagaagggcactgaactgttccagggcctgctccagttgagccacttggcctgagaattcctgctccgaaagggccatctggctgaccaggttctccaaacagctctgcgtttggaatacactgtcttcccactgcttccagtcggcacgcagggcctgcatctccgtgtgcatgagctcacacccactggcagttgtgttctgtttcacttcgggagccagcgactccactctgctgagacggcttgcaccaatctctctggaatctatcagctccttaatttttgataactttttctgggtggctgatgaatctccagacatatctgaccaccggtgaagttcttcctttgctgaatggagccaatctgtgaactcgtggaccgcatctaaatacattagatgatctttcacaatctcttccactttcctcattttttccttggcaacagtcattatatcattaaactgtgttttcagctcctcttgagctgtgtccttgaaagactcatcctctgtcttttcgtagagctccctggacttcgcaattagacggtgaagggctctcgtgtgatcttctgcctcagacaggatggactggaggtggtcaagcaggacgaacttctctttcagacctggctgtggttgtaagggatgttctattttttgatccactgattccatccactgctccaactggtttttcctctctacatagtcattccattggctaatcacagactctaaagtgctttgagcgtggacggaggagctcatgatgtcagcccacacttctttaagggtctctaactgagtctgaatcaccctctgaccttctttgttgctacttctcaaggcctgttcccccttgccaatggccatattcaacttaacttccccttcacctttcatcaggagaatatcctgtatttgtgacagccgtttctccagggtgtctttgctcccaagagtgctctctgcacaggccagtctgtcctgaatggccttcacccagaaccacatgctttgcagtgcttcctccagggcttcgtgctcctgaagggccacctggcagctccggagtttctctttggtcattctaagtaggttctggtggcttgtgaggagctgggaacacaggcggccctcctgcccagcaccgtggccttcttcactcagaagctgccctctctgggaaagcttatcaagagactctcttgcagccagcagttctcccaaaaacatttcaactttatgaacttcatttttcttctcaggaatgtgctgtttactctctcccaagttttccgtattgaacctttcttccatttcatggatccataagttcagttttctgtgctgatcttcaaagcttccaagttctgaagcacagtcttgaagagcctgcttatctttaaggcattgtttcagaaatgcttgaaactcttcattggcctttgtgatttgttcttgaatgctactgacaatttgtttagacaaatgtgcatacaaagtttgtccttcttgagtcactgcatcaagtttgctctgcccatcactgactgagtccaaaatgttctgaagatcatggagctttgcttctagaactttgctgtcaccggtgcgatctgatgattcttttgctgctgcctttgctcccaaaaaccattcttggaattcctgcatagactcactgaagtgtttttccagagattcctgcaggctggcctgggttttggagcacaactggctcacggcttcatgtttctttatcagaccagtcattgcacggcccaggctctccaactcagctgagtggtacttgcggcacaagctattgagattttcttgggtagagctgatgttgctttgttgactttgaagttctttttgtatatccttgacttttttcaatgcttcacaagtctcattttgggcacagttcatcaacgattcttccacttttgtgaaccatgttgttatgtcattaataaacttctccacttgtgtactttgagccgtgaaatccttcagggttccttttgctacttcagttatttctttggcatgctccagtttctgcattaagtctgcttctataaactgaaggtctggcggtgtttctagatttttagttaattctttcagatcattaactttggaatgcagttcttccaatctcaatgctttgtttttaacttcagactcaaattctttaagcagttcttcagctctgaggtggttatccaggttgctgatgttttctgccatctgtggaacgcagttgtttgaccatccctcaatctcatctctagttgacagtacatcatcccaaatggacaggcttactctcagcctatccatgttttcttcaagtttctctgatacatccagccatttgtccacggtgctctccatgtctgttttcaccaagctgaaatcactactgtgaattttcttcagctcagataacaagtgttttcctttgctggtaaagttatccaagtctttctgtttgtaattcattttgttcttggcagtttcatgcttggaaaaagcccatttaagatcctcctgatcttttatggtagttctggttacaatcacactgctggcattttctaagactttagatacagctgatttcaggttctgatattctctcattaagtcaataagtccacagcactgaccctgattttcatgaattagtcttttggtatcatcccaggtgacctctaagcggtttatctccctgtcaacttcaggtgcaaaagctacatctttctgggcaatttgcttggctttgtctttcaaccaacatagttcatgctcgtgagaattcaattcatcttctagctgattaaacactcttaacctctgctgaagagcttggcgggtaggttctttcaatcgctctttgtcagtcctttcttcaatgtcctcaatgcttttcagaagctcctctttctggtcttggaatgcttttttcaacactgccagagcatctgcctcactctgcttggttcccagaaggttctggatcctctctacctctccacagagctgatcagccgtggctctgcaggaagtcctttgctcagagctcccgattttcagatggtattgggctttggaaagaatgccatccagactgacggcagcagattctaatgctttagcattttgaagagcatcattgaggtccttttctatcaaatcagactcgttcttattcatactgttggttgcttccactgtttgcctcagctggcggagaatgccggacagagaggcatggctctggaggaattctgccaaatgggacagggcaagctgccgcctctccacaacctggctggcctcctcaaacagctggaagcagtcctcagcctttccctgcaggaggtggaggtcctcagcacggcccagagaacccaactttgctaagtgaccctgcagactctgcaattcgccctttttgctctctacttctgctgcgtggtccttatgccgagtaagggctacttgatggtccattatgctaatctcagaggtagtttgtaattcactgagaaacagtttaatccagacagaaaaggaaagcagcagctcatcaaattgctggtgttcagcaaccacagactgaagaaaattaatccttttgttaatgatctgtggtaaatctctccatctctcatccaactgctccaaatgtagtttcatcattttcacatcatctttggaggctactgagaacaatgattccttcaattgcaaaagtttgctatagaatgaggcctgggatacaacttcattttgcagtgcctgtattaactgaagttcaccttccactttgactctgtctgcagaaatgtccatttctggggaactggctttagcttcaccccgctctaaccaggtcaaaaaggatgatagttctttctctagcctctgccagtgggccagcagattctccagcgccgtctgtctctccttcgccctccttaggatgtcctcgtattgctgctgtagagccgcagcctcctgaacacaggaatctctgttcacaaccttcctggcactggctgagaaggcagtgatcgcgctgctcagtgactccagggcctggcagagatccatatgttcttgaagaactttgtatgtttctgtagctgaagaacatattttaattggaacagcaagtttatcttcaaattcagacacagattgctggatctttctaaggttctcttcaaacttttgctgctgagataaatgtcccaggattgttccttccagacactgtgcatgctctcgaagctcttccccgtatcttcttatttgtgtcaacttggctttaattcgagcagattctccagtggtaacaaactgagcaaaagactgggcttcttcttctaatcctacaatgctgctgagcttactttctatttcctgaattgtgaccttaatttggctgatttgcatgtccatggcagatgacgaagtttccaaggcattgagttctttttctttctcagttatccagacggacagagtctcaaaattactgccaaaatgatcccacttggttttcaccatttccatggttttaatatcttcttcaagcgtgtcttctaattttttgacttgttctttgattgacttggcctgctgttgaagcagctgcttattttggggcccaagcggtatctctgaagcttcctttacaaggttctcagcctggactgcaatactttctgtccgtttagaaaactcctttgtttgttccagttctgaagataaactttccaaactgctaaaactcaagaagcgttcatgactggaacctgtttgaaaaaggtatcttactactgtttctttgtttgtttcaaatcgctcccattttcttaatgtgacctggatgcggcgttcctgcctctcccggctgcgctccaggccatccagtgtgctctccagcttccgcagctcctcgtggcctcggtcaggcagccccccttctccctgctgcgcctgcgcgatctgctgctgcacatctctcttctttgctgagatccgctttgtcttttgctggtgatgaagaagtaactgctgtgcttcaaacagattttcagtatccaagatcttctcagcttgttcctggacttctttagagccagaaattaattcttcgagagaatttttgactatttctttgtactggacacagtccccaaaattgcttagcatcttttcaacctctgacagcagcgtcacaagagccttgaaagagctggataattttgccagctcatctccctgcttttgggcttcattctcagaagaaacttctgtcaaaactttcagcctggatttcagccagctgagggtctcaccccttttggtaacaccatttctgatctcttcaacggcacgtttaacctctccgtggttggcagtatcgatggcctcacccttgatcccctttaattgtgtctcatttgtagatatccaagatgagaactcagagaatctgctagtgtagtccttccacttgtctgggtcttccatgagcttcctgtaggtgctgtcaatggcagctctgagctctttgagagtcacgtgacaggttccaggtgtgtcccttactgggtcccgcactgggagtttcacacagagttcctcgatgagctgtaaccttttctcacagagatgatgaggacctttgtcactgaagaaaaccctgtgctctttaattatcttttcactgccttcctggggcatcagcttggtctctcgatccagctcagttctgcattcttctacagaggctaagaacctattcttctccacatcaatcttcagatgaagcaaatgataaggggcttctccttgaagatccttccattgtttgtggagctttcgaacagcttcctgcagcccctgctgctcctgctctggaaggatgtcggtgagttcatcacaagctttcaggaaagcattgagcaccctctgatccagctgactgaaaaactcagtgtgtctccgcaggagctcctctggatcccccttttcctccaggccctcctgagcaatccgcagtaccttctccaactctgctcgagactcctcaaacttcttcatcaagcgactgttggtttccacatgcttcttccaatctccagttttctttaccatactctgaaaagcaacatgaatatctgcaatctgtctttgtagcctcgtctgatcaaaatgctttaacacgttgctcaaggtcacaaacttttgaacactttgactgcctttctcaataagtgtcaaggttttcttacagttttcttgacaagctaacagttcctgatgtttttgtttaaaaagggcactcgattgtgcctcacgctcaagaactgtgataatttcattgattttcccaagtgagtcataaaaggacgtcatctgcttttctaattcctccaacggaatcaacagctgctgagactcataaaggagtggggagtaacattctttgaccttggttagctgctctttgagctttgacatggtcgcaaacatttcttttccttcttcttgggggctttctttggtaatgaggtgtgctgtctttgtaattatcttgtattgggcatccatcacaggcaccctctgctcaatatcctccaagtcttgaattaatagcttgacattcataaaagagacttctaagggttcagaaagtttcttatgggcttccgttgcaaaagcagacagggtaacaacacagtctgtgtattccttcttcattctgtccatctcatcagcttgagcatattgcttgacttccataaacaactccctccaccgcccatttagcaacagtaattgctgcttcaggtcacgggaaaccatctcatcacaggtttcaattagaaaattgccagcatcgttcatggcagtatgctgctgaatccaatgaggtaaatttcgaaaaaaatcctttttggcattttctgattgattgagcattttttcagcatcctctagccaggcttgcagactagccactgtattgccatagcgatcccagttagagatcacttcttccagcatgctcctcacactcctcacttctactgagagattcctccactgagcggtggtttcattcatgaatttcatcacattctcagcttcttccactgaaccatctgctttgacatacatctcagctgtctgtttcaagatctggtatgtcacctcatattgttcaaagaacttgctattttctataaaagacacgtagttttgtagaagctgctccactgactctctcctcccgtacttaatgatccaagacttcagctttgactctgttacatgtcagccttaaatagaatgcagccacaagctcttctaactctggctgatcattttctggaaatccgattccttttctagctctggatttaaaagcaaagcatgaatgattgaagtcttcgatttagttcttt

SEQ ID NO: 9579 - RNA, 12288 nt, Homo sapiens
  source 1..12288: mol_type = other RNA
agttcttcagtggcaagctttatcaaaatcttccttaaaatgcttcctagaaaccaaattcttctctagttcttgtaaccggtgactgcacttttgtaaaacactgtcatagacactctgcaattcctgaagcttccccagcacttcactcttttcctgctctgtgacttccttcattagttcgcgaccctgggcccaaagtccagtgacttcattttggtaagtcttgaggctggcttgtgcactcttacatgttttgacttgtttgctcacatcatctggtaacagacagatgtgttcacggaacattatctttcgctcatgttgctgaatttggctggtggcctggaacactgccatgagaaactgggttttctcggacaaggctttgtttaagtactttcttcgctggcccactaagtcactgagacaattcacgtggctttgtgcatcagagagagccttctggatgacctgtcgctcattgagaccaagatctgccatgaccctgtctgcgtcctttataagcgatttcaggagcatctgcttggcctccagttcactgcagatggccaggtgatccatgagaaggttctgagccatatctggaggagggctctgcttaagggcctcggcgatgttgggttgttgctcttctgcccactccattagctcctgaaatctggactgcaccacatttaactcctccaagttggtgactgacacttggattttccttttaatgaggtcctcaagctgaaaccaacgttgctctaaatgactcgtctgttctttgactaactccttgtcatctaaattcagatgctctatcattttctgcttttgatctttcagatcttcaatagcatactttctctcctgcaatgccaatgctaactttttcaaagcttccaggtggacagctgtactctctgcatcagatctggccaagttatcccattctgtagtaaatttttctaggaacacttcaacaacattcatacagtcatggtaatctcttgttctctgaagatcctcttccctttgcaagcacaggttgttagactgacggcacaaatcgagccactgatcatttaaatgatttatttccttgtgttcaggcgattcctccttctttgttaacttattcaccttttctattatggtgttcacggatgcctgtttgctctgtagtttcttaacaaaatccttaacttgtgaaaccatgttctgtgcaatgttcagctccagctcagagtgcctcctcttcatgttctgcagttgctgatcagcatcttgcaggtaaatccagagctcagacttcaggtgcttgatctcttcccagccctgagttaagttctgggcctggacaagcttttgttcaatcgtttgctctgtttgttgaatgtcttttgctgtggttttcaccgaagcatttgacaggtcacacatggagcaaaggagatctaggtaggtccttgcctgctcttgcaaagctctgaagtgtttgacctgcttaatggcttctgccctactaagaggtggttgaggacttggctctaaatccggctggactgcagaaagccaggcctggcactgctgcagggtgtcttgtcggctgacgtgcttctgaagttcgtgttccaaactctggtacatcctctgagctgtgctgcagatcgctgagtagctgtcctttgtgccctgcagatgagcatgcacgttttgtttaagtttcgcttgcaggtggtctgcacattggccaatcaaagtatcacctttcatttgaagattgttcaaacggtcttcaaaaccagcaatttcttccatcattgccttgtggtgggccaattgctgggtgattgtctccaggctgcttgtctccaggaggtcaggtgccaccagtctgccagacatctgcagcagccacttttcgacctcttggagctcactgttgtagtcttcatggtctttgactttcgcctccagactgaagacatgctcctttcctatgctgcacaggtcctggtaatcactttgaagttgatctattttgtcctttaaagtgacgtcctgcaccagttccaaaagagcttcacccttctctctcactgactttactgatggttcatgggacagcaccgtttgttgaagtgacttgtatttagataactgagcttttttctcatataattccattttgggttcttcaggaacatgtagaatttcctggtattctgctatccactgtgtcagtgctttgcatttatctgagaattcctttgctaaatgaagacctttttccagcgtcatgtgttctttccggacagtgctggtcagttccttcaactgctccatgtgatcatgaatctcctttcttaacctctctgcctcgccttcctccaagtatttaacagccctctctcctttctcccgggctgatttcagcaaactgtgacctttctccatgtctttgagcaaaacctccaacgtcttcaatttcttccccatcattactgtatctactttgtcaatcttggtagccacattcttgaagtttttatgagtagagccataccaatcagaataggaactgagggatgattctgattcctccaaactctgaatctcctcctccaggaattttatttgttccagcacttggagaagcagggcctggtatctggaagtcagctgggtggcctggcaacccattctgctgttcacgtggctctcgtccagtatctcctgagctctagctcccacttcctcaacttcatctctgtatgcagtcacttcttcgtgccacttcttcatctgatgtaattgtatctccttggttgccctgttagactgacgtctggtcctgggactaactttctcctctgctgttttgagccattcatctacttgctgaaacttttgctccattagcctcaatttgttcaccacgttattgaactgagttcgagtctcggacagcctgtgctggtaagcctgccagtcttgccggagagactctaaagcccggtcctctgcctgtgggatacctgatgggatcacatcctctctggtgtgcagcactgagttcaacagggcctgcccctctgcacagtgtacctgtagctcctgaagatcacgcaatgttgtctcatgagtgtgggcatcaccttcaagaactgaatactggtcgagcttttcttgttcttgccccaaccaaacttcaaatgcctttaggtctctctgatactcttggtgcaggcggacaagtttttcagacttggttacggcttccttggccctctcttggatggctctgtatcgttcctgtagatcctggagttctagctgggtgacatagtgttctgtcatgccagcccctttgacttcgatggtctccagcaagctgctgtaactcagcacttcttcatttaataacttggcttttccgagcatcgttgttttatcccgcagctccgcatgctgcctttctgattcattcaggttggcttccatactatccatccaaccggagaactgtcgaacgccatcctgataacttgtccacttggagagagctccttcgagttggcttttacaacgaatccctgcagacaaaagggatgcccacatatccttcacactctgcagctgctgctgaatagtgggaatgccttctggagaagtattctgaaggacagattctcccctggtcactatcattttcatctgaatctctttttcctgtttgactgataatagagcctcgagcttgagcgtcctgctgtccagcacacttttgtcggatgtcgggtggcagtatgaatccagcatgtgaatcgcatccgtcatccagtcttgtaattctttaatcccaagagagaactgattgtgttctgcaacgattctatccagtcttgacactttctcctttgttaaattgcttagcgctagatactgagaagacagctgcgacactctgtgcctaaagctcttgctggcagcttgtccttcccacagctgctgagctttctctttcagcctgttgagctgaggctcgtagcagtgtatttcctcaaggacagactggagcttctgctgctccctcctctttgctggcagatcatagaggcgattgctgctttcatggaccatcttctcagttttactcagccagtcctggataggctcagcacttacttcaaagtccttcatttggatctttagattctctagagcagattctttttggtggagatttgaatgaaaatttttccaatcttcttttgcagctgtaactttggcctggatccctttcgctttctctttggtcagcagggtactcagaagttcccctttagacagcatcatgtttagcttgtgctgtccattttcactttctgacaaaaactcctgtattttctgaagactagttgaaacttcacttatattttgaggtatatcaaaacacttggcggtagtgatttttgcattaaccaaccactgctggaaatccctgaaggcctttcgaaatctttgctgtaaaatctgttctttattctggcagcccttggatgcttgcaaacaaagacaattatactctttaatcaagccagaaacttttccactgtaggtactcaggtctctggaaaatcgacaaagttcattcagctgagacttgagatcctctgttctaggctctgctttttgcaaagcatccagtatctcttgtcctttgtgccagcattccactatctcctcatccgtgttcttgccttccaggagggttaactgctgagcccaggttttcagaagggcactgaactgttccagggcctgctccagttgagccacttggcctgagaattcctgctccgaaagggccatctggctgaccaggttctccaaacagctctgcgtttggaatacactgtcttcccactgcttccagtcggcacgcagggcctgcatctccgtgtgcatgagctcacacccactggcagttgtgttctgtttcacttcgggagccagcgactccactctgctgagacggcttgcaccaatctctctggaatctatcagctccttaatttttgataactttttctgggtggctgatgaatctccagacatatctgaccaccggtgaagttcttcctttgctgaatggagccaatctgtgaactcgtggaccgcatctaaatacattagatgatctttcacaatctcttccactttcctcattttttccttggcaacagtcattatatcattaaactgtgttttcagctcctcttgagctgtgtccttgaaagactcatcctctgtcttttcgtagagctccctggacttcgcaattagacggtgaagggctctcgtgtgatcttctgcctcagacaggatggactggaggtggtcaagcaggacgaacttctctttcagacctggctgtggttgtaagggatgttctattttttgatccactgattccatccactgctccaactggtttttcctctctacatagtcattccattggctaatcacagactctaaagtgctttgagcgtggacggaggagctcatgatgtcagcccacacttctttaagggtctctaactgagtctgaatcaccctctgaccttctttgttgctacttctcaaggcctgttcccccttgccaatggccatattcaacttaacttccccttcacctttcatcaggagaatatcctgtatttgtgacagccgtttctccagggtgtctttgctcccaagagtgctctctgcacaggccagtctgtcctgaatggccttcacccagaaccacatgctttgcagtgcttcctccagggcttcgtgctcctgaagggccacctggcagctccggagtttctctttggtcattctaagtaggttctggtggcttgtgaggagctgggaacacaggcggccctcctgcccagcaccgtggccttcttcactcagaagctgccctctctgggaaagcttatcaagagactctcttgcagccagcagttctcccaaaaacatttcaactttatgaacttcatttttcttctcaggaatgtgctgtttactctctcccaagttttccgtattgaacctttcttccatttcatggatccataagttcagttttctgtgctgatcttcaaagcttccaagttctgaagcacagtcttgaagagcctgcttatctttaaggcattgtttcagaaatgcttgaaactcttcattggcctttgtgatttgttcttgaatgctactgacaatttgtttagacaaatgtgcatacaaagtttgtccttcttgagtcactgcatcaagtttgctctgcccatcactgactgagtccaaaatgttctgaagatcatggagctttgcttctagaactttgctgtcaccggtgcgatctgatgattcttttgctgctgcctttgctcccaaaaaccattcttggaattcctgcatagactcactgaagtgtttttccagagattcctgcaggctggcctgggttttggagcacaactggctcacggcttcatgtttctttatcagaccagtcattgcacggcccaggctctccaactcagctgagtggtacttgcggcacaagctattgagattttcttgggtagagctgatgttgctttgttgactttgaagttctttttgtatatccttgacttttttcaatgcttcacaagtctcattttgggcacagttcatcaacgattcttccacttttgtgaaccatgttgttatgtcattaataaacttctccacttgtgtactttgagccgtgaaatccttcagggttccttttgctacttcagttatttctttggcatgctccagtttctgcattaagtctgcttctataaactgaaggtctggcggtgtttctagatttttagttaattctttcagatcattaactttggaatgcagttcttccaatctcaatgctttgtttttaacttcagactcaaattctttaagcagttcttcagctctgaggtggttatccaggttgctgatgttttctgccatctgtggaacgcagttgtttgaccatccctcaatctcatctctagttgacagtacatcatcccaaatggacaggcttactctcagcctatccatgttttcttcaagtttctctgatacatccagccatttgtccacggtgctctccatgtctgttttcaccaagctgaaatcactactgtgaattttcttcagctcagataacaagtgttttcctttgctggtaaagttatccaagtctttctgtttgtaattcattttgttcttggcagtttcatgcttggaaaaagcccatttaagatcctcctgatcttttatggtagttctggttacaatcacactgctggcattttctaagactttagatacagctgatttcaggttctgatattctctcattaagtcaataagtccacagcactgaccctgattttcatgaattagtcttttggtatcatcccaggtgacctctaagcggtttatctccctgtcaacttcaggtgcaaaagctacatctttctgggcaatttgcttggctttgtctttcaaccaacatagttcatgctcgtgagaattcaattcatcttctagctgattaaacactcttaacctctgctgaagagcttggcgggtaggttctttcaatcgctctttgtcagtcctttcttcaatgtcctcaatgcttttcagaagctcctctttctggtcttggaatgcttttttcaacactgccagagcatctgcctcactctgcttggttcccagaaggttctggatcctctctacctctccacagagctgatcagccgtggctctgcaggaagtcctttgctcagagctcccgattttcagatggtattgggctttggaaagaatgccatccagactgacggcagcagattctaatgctttagcattttgaagagcatcattgaggtccttttctatcaaatcagactcgttcttattcatactgttggttgcttccactgtttgcctcagctggcggagaatgccggacagagaggcatggctctggaggaattctgccaaatgggacagggcaagctgccgcctctccacaacctggctggcctcctcaaacagctggaagcagtcctcagcctttccctgcaggaggtggaggtcctcagcacggcccagagaacccaactttgctaagtgaccctgcagactctgcaattcgccctttttgctctctacttctgctgcgtggtccttatgccgagtaagggctacttgatggtccattatgctaatctcagaggtagtttgtaattcactgagaaacagtttaatccagacagaaaaggaaagcagcagctcatcaaattgctggtgttcagcaaccacagactgaagaaaattaatccttttgttaatgatctgtggtaaatctctccatctctcatccaactgctccaaatgtagtttcatcattttcacatcatctttggaggctactgagaacaatgattccttcaattgcaaaagtttgctatagaatgaggcctgggatacaacttcattttgcagtgcctgtattaactgaagttcaccttccactttgactctgtctgcagaaatgtccatttctggggaactggctttagcttcaccccgctctaaccaggtcaaaaaggatgatagttctttctctagcctctgccagtgggccagcagattctccagcgccgtctgtctctccttcgccctccttaggatgtcctcgtattgctgctgtagagccgcagcctcctgaacacaggaatctctgttcacaaccttcctggcactggctgagaaggcagtgatcgcgctgctcagtgactccagggcctggcagagatccatatgttcttgaagaactttgtatgtttctgtagctgaagaacatattttaattggaacagcaagtttatcttcaaattcagacacagattgctggatctttctaaggttctcttcaaacttttgctgctgagataaatgtcccaggattgttccttccagacactgtgcatgctctcgaagctcttccccgtatcttcttatttgtgtcaacttggctttaattcgagcagattctccagtggtaacaaactgagcaaaagactgggcttcttcttctaatcctacaatgctgctgagcttactttctatttcctgaattgtgaccttaatttggctgatttgcatgtccatggcagatgacgaagtttccaaggcattgagttctttttctttctcagttatccagacggacagagtctcaaaattactgccaaaatgatcccacttggttttcaccatttccatggttttaatatcttcttcaagcgtgtcttctaattttttgacttgttctttgattgacttggcctgctgttgaagcagctgcttattttggggcccaagcggtatctctgaagcttcctttacaaggttctcagcctggactgcaatactttctgtccgtttagaaaactcctttgtttgttccagttctgaagataaactttccaaactgctaaaactcaagaagcgttcatgactggaacctgtttgaaaaaggtatcttactactgtttctttgtttgtttcaaatcgctcccattttcttaatgtgacctggatgcggcgttcctgcctctcccggctgcgctccaggccatccagtgtgctctccagcttccgcagctcctcgtggcctcggtcaggcagccccccttctccctgctgcgcctgcgcgatctgctgctgcacatctctcttctttgctgagatccgctttgtcttttgctggtgatgaagaagtaactgctgtgcttcaaacagattttcagtatccaagatcttctcagcttgttcctggacttctttagagccagaaattaattcttcgagagaatttttgactatttctttgtactggacacagtccccaaaattgcttagcatcttttcaacctctgacagcagcgtcacaagagccttgaaagagctggataattttgccagctcatctccctgcttttgggcttcattctcagaagaaacttctgtcaaaactttcagcctggatttcagccagctgagggtctcaccccttttggtaacaccatttctgatctcttcaacggcacgtttaacctctccgtggttggcagtatcgatggcctcacccttgatcccctttaattgtgtctcatttgtagatatccaagatgagaactcagagaatctgctagtgtagtccttccacttgtctgggtcttccatgagcttcctgtaggtgctgtcaatggcagctctgagctctttgagagtcacgtgacaggttccaggtgtgtcccttactgggtcccgcactgggagtttcacacagagttcctcgatgagctgtaaccttttctcacagagatgatgaggacctttgtcactgaagaaaaccctgtgctctttaattatcttttcactgccttcctggggcatcagcttggtctctcgatccagctcagttctgcattcttctacagaggctaagaacctattcttctccacatcaatcttcagatgaagcaaatgataaggggcttctccttgaagatccttccattgtttgtggagctttcgaacagcttcctgcagcccctgctgctcctgctctggaaggatgtcggtgagttcatcacaagctttcaggaaagcattgagcaccctctgatccagctgactgaaaaactcagtgtgtctccgcaggagctcctctggatcccccttttcctccaggccctcctgagcaatccgcagtaccttctccaactctgctcgagactcctcaaacttcttcatcaagcgactgttggtttccacatgcttcttccaatctccagttttctttaccatactctgaaaagcaacatgaatatctgcaatctgtctttgtagcctcgtctgatcaaaatgctttaacacgttgctcaaggtcacaaacttttgaacactttgactgcctttctcaataagtgtcaaggttttcttacagttttcttgacaagctaacagttcctgatgtttttgtttaaaaagggcactcgattgtgcctcacgctcaagaactgtgataatttcattgattttcccaagtgagtcataaaaggacgtcatctgcttttctaattcctccaacggaatcaacagctgctgagactcataaaggagtggggagtaacattctttgaccttggttagctgctctttgagctttgacatggtcgcaaacatttcttttccttcttcttgggggctttctttggtaatgaggtgtgctgtctttgtaattatcttgtattgggcatccatcacaggcaccctctgctcaatatcctccaagtcttgaattaatagcttgacattcataaaagagacttctaagggttcagaaagtttcttatgggcttccgttgcaaaagcagacagggtaacaacacagtctgtgtattccttcttcattctgtccatctcatcagcttgagcatattgcttgacttccataaacaactccctccaccgcccatttagcaacagtaattgctgcttcaggtcacgggaaaccatctcatcacaggtttcaattagaaaattgccagcatcgttcatggcagtatgctgctgaatccaatgaggtaaatttcgaaaaaaatcctttttggcattttctgattgattgagcattttttcagcatcctctagccaggcttgcagactagccactgtattgccatagcgatcccagttagagatcacttcttccagcatgctcctcacactcctcacttctactgagagattcctccactgagcggtggtttcattcatgaatttcatcacattctcagcttcttccactgaaccatctgctttgacatacatctcagctgtctgtttcaagatctggtatgtcacctcatattgttcaaagaacttgctattttctataaaagacacgtagttttgtagaagctgctccactgactctctcctcccgtacttaatgatccaagacttcagctttgactttaacctgttacatgtcagccttaaatagaatgcagccacaagctcttctaactctggctgatcattttctggaaatccgattccttttctagctctggatttaaaagc

SEQ ID NO: 9580 - RNA, 14078 nt, Homo sapiens
  source 1..14078: mol_type = other RNA
agttcttcagtggcaagctttatcaaaatcttccttaaaatgcttcctagaaaccaaattcttctctagttcttgtaaccggtgactgcacttttgtaaaacactgtcatagacactctgcaattcctgaagcttccccagcacttcactcttttcctgctctgtgacttccttcattagttcgcgaccctgggcccaaagtccagtgacttcattttggtaagtcttgaggctggcttgtgcactcttacatgttttgacttgtttgctcacatcatctggtaacagacagatgtgttcacggaacattatctttcgctcatgttgctgaatttggctggtggcctggaacactgccatgagaaactgggttttctcggacaaggctttgtttaagtactttcttcgctggcccactaagtcactgagacaattcacgtggctttgtgcatcagagagagccttctggatgacctgtcgctcattgagaccaagatctgccatgaccctgtctgcgtcctttataagcgatttcaggagcatctgcttggcctccagttcactgcagatggccaggtgatccatgagaaggttctgagccatatctggaggagggctctgcttaagggcctcggcgatgttgggttgttgctcttctgcccactccattagctcctgaaatctggactgcaccacatttaactcctccaagttggtgactgacacttggattttccttttaatgaggtcctcaagctgaaaccaacgttgctctaaatgactcgtctgttctttgactaactccttgtcatctaaattcagatgctctatcattttctgcttttgatctttcagatcttcaatagcatactttctctcctgcaatgccaatgctaactttttcaaagcttccaggtggacagctgtactctctgcatcagatctggccaagttatcccattctgtagtaaatttttctaggaacacttcaacaacattcatacagtcatggtaatctcttgttctctgaagatcctcttccctttgcaagcacaggttgttagactgacggcacaaatcgagccactgatcatttaaatgatttatttccttgtgttcaggcgattcctccttctttgttaacttattcaccttttctattatggtgttcacggatgcctgtttgctctgtagtttcttaacaaaatccttaacttgtgaaaccatgttctgtgcaatgttcagctccagctcagagtgcctcctcttcatgttctgcagttgctgatcagcatcttgcaggtaaatccagagctcagacttcaggtgcttgatctcttcccagccctgagttaagttctgggcctggacaagcttttgttcaatcgtttgctctgtttgttgaatgtcttttgctgtggttttcaccgaagcatttgacaggtcacacatggagcaaaggagatctaggtaggtccttgcctgctcttgcaaagctctgaagtgtttgacctgcttaatggcttctgccctactaagaggtggttgaggacttggctctaaatccggctggactgcagaaagccaggcctggcactgctgcagggtgtcttgtcggctgacgtgcttctgaagttcgtgttccaaactctggtacatcctctgagctgtgctgcagatcgctgagtagctgtcctttgtgccctgcagatgagcatgcacgttttgtttaagtttcgcttgcaggtggtctgcacattggccaatcaaagtatcacctttcatttgaagattgttcaaacggtcttcaaaaccagcaatttcttccatcattgccttgtggtgggccaattgctgggtgattgtctccaggctgcttgtctccaggaggtcaggtgccaccagtctgccagacatctgcagcagccacttttcgacctcttggagctcactgttgtagtcttcatggtctttgactttcgcctccagactgaagacatgctcctttcctatgctgcacaggtcctggtaatcactttgaagttgatctattttgtcctttaaagtgacgtcctgcaccagttccaaaagagcttcacccttctctctcactgactttactgatggttcatgggacagcaccgtttgttgaagtgacttgtatttagataactgagcttttttctcatataattccattttgggttcttcaggaacatgtagaatttcctggtattctgctatccactgtgtcagtgctttgcatttatctgagaattcctttgctaaatgaagacctttttccagcgtcatgtgttctttccggacagtgctggtcagttccttcaactgctccatgtgatcatgaatctcctttcttaacctctctgcctcgccttcctccaagtatttaacagccctctctcctttctcccgggctgatttcagcaaactgtgacctttctccatgtctttgagcaaaacctccaacgtcttcaatttcttccccatcattactgtatctactttgtcaatcttggtagccacattcttgaagtttttatgagtagagccataccaatcagaataggaactgagggatgattctgattcctccaaactctgaatctcctcctccaggaattttatttgttccagcacttggagaagcagggcctggtatctggaagtcagctgggtggcctggcaacccattctgctgttcacgtggctctcgtccagtatctcctgagctctagctcccacttcctcaacttcatctctgtatgcagtcacttcttcgtgccacttcttcatctgatgtaattgtatctccttggttgccctgttagactgacgtctggtcctgggactaactttctcctctgctgttttgagccattcatctacttgctgaaacttttgctccattagcctcaatttgttcaccacgttattgaactgagttcgagtctcggacagcctgtgctggtaagcctgccagtcttgccggagagactctaaagcccggtcctctgcctgtgggatacctgatgggatcacatcctctctggtgtgcagcactgagttcaacagggcctgcccctctgcacagtgtacctgtagctcctgaagatcacgcaatgttgtctcatgagtgtgggcatcaccttcaagaactgaatactggtcgagcttttcttgttcttgccccaaccaaacttcaaatgcctttaggtctctctgatactcttggtgcaggcggacaagtttttcagacttggttacggcttccttggccctctcttggatggctctgtatcgttcctgtagatcctggagttctagctgggtgacatagtgttctgtcatgccagcccctttgacttcgatggtctccagcaagctgctgtaactcagcacttcttcatttaataacttggcttttccgagcatcgttgttttatcccgcagctccgcatgctgcctttctgattcattcaggttggcttccatactatccatccaaccggagaactgtcgaacgccatcctgataacttgtccacttggagagagctccttcgagttggcttttacaacgaatccctgcagacaaaagggatgcccacatatccttcacactctgcagctgctgctgaatagtgggaatgccttctggagaagtattctgaaggacagattctcccctggtcactatcattttcatctgaatctctttttcctgtttgactgataatagagcctcgagcttgagcgtcctgctgtccagcacacttttgtcggatgtcgggtggcagtatgaatccagcatgtgaatcgcatccgtcatccagtcttgtaattctttaatcccaagagagaactgattgtgttctgcaacgattctatccagtcttgacactttctcctttgttaaattgcttagcgctagatactgagaagacagctgcgacactctgtgcctaaagctcttgctggcagcttgtccttcccacagctgctgagctttctctttcagcctgttgagctgaggctcgtagcagtgtatttcctcaaggacagactggagcttctgctgctccctcctctttgctggcagatcatagaggcgattgctgctttcatggaccatcttctcagttttactcagccagtcctggataggctcagcacttacttcaaagtccttcatttggatctttagattctctagagcagattctttttggtggagatttgaatgaaaatttttccaatcttcttttgcagctgtaactttggcctggatccctttcgctttctctttggtcagcagggtactcagaagttcccctttagacagcatcatgtttagcttgtgctgtccattttcactttctgacaaaaactcctgtattttctgaagactagttgaaacttcacttatattttgaggtatatcaaaacacttggcggtagtgatttttgcattaaccaaccactgctggaaatccctgaaggcctttcgaaatctttgctgtaaaatctgttctttattctggcagcccttggatgcttgcaaacaaagacaattatactctttaatcaagccagaaacttttccactgtaggtactcaggtctctggaaaatcgacaaagttcattcagctgagacttgagatcctctgttctaggctctgctttttgcaaagcatccagtatctcttgtcctttgtgccagcattccactatctcctcatccgtgttcttgccttccaggagggttaactgctgagcccaggttttcagaagggcactgaactgttccagggcctgctccagttgagccacttggcctgagaattcctgctccgaaagggccatctggctgaccaggttctccaaacagctctgcgtttggaatacactgtcttcccactgcttccagtcggcacgcagggcctgcatctccgtgtgcatgagctcacacccactggcagttgtgttctgtttcacttcgggagccagcgactccactctgctgagacggcttgcaccaatctctctggaatctatcagctccttaatttttgataactttttctgggtggctgatgaatctccagacatatctgaccaccggtgaagttcttcctttgctgaatggagccaatctgtgaactcgtggaccgcatctaaatacattagatgatctttcacaatctcttccactttcctcattttttccttggcaacagtcattatatcattaaactgtgttttcagctcctcttgagctgtgtccttgaaagactcatcctctgtcttttcgtagagctccctggacttcgcaattagacggtgaagggctctcgtgtgatcttctgcctcagacaggatggactggaggtggtcaagcaggacgaacttctctttcagacctggctgtggttgtaagggatgttctattttttgatccactgattccatccactgctccaactggtttttcctctctacatagtcattccattggctaatcacagactctaaagtgctttgagcgtggacggaggagctcatgatgtcagcccacacttctttaagggtctctaactgagtctgaatcaccctctgaccttctttgttgctacttctcaaggcctgttcccccttgccaatggccatattcaacttaacttccccttcacctttcatcaggagaatatcctgtatttgtgacagccgtttctccagggtgtctttgctcccaagagtgctctctgcacaggccagtctgtcctgaatggccttcacccagaaccacatgctttgcagtgcttcctccagggcttcgtgctcctgaagggccacctggcagctccggagtttctctttggtcattctaagtaggttctggtggcttgtgaggagctgggaacacaggcggccctcctgcccagcaccgtggccttcttcactcagaagctgccctctctgggaaagcttatcaagagactctcttgcagccagcagttctcccaaaaacatttcaactttatgaacttcatttttcttctcaggaatgtgctgtttactctctcccaagttttccgtattgaacctttcttccatttcatggatccataagttcagttttctgtgctgatcttcaaagcttccaagttctgaagcacagtcttgaagagcctgcttatctttaaggcattgtttcagaaatgcttgaaactcttcattggcctttgtgatttgttcttgaatgctactgacaatttgtttagacaaatgtgcatacaaagtttgtccttcttgagtcactgcatcaagtttgctctgcccatcactgactgagtccaaaatgttctgaagatcatggagctttgcttctagaactttgctgtcaccggtgcgatctgatgattcttttgctgctgcctttgctcccaaaaaccattcttggaattcctgcatagactcactgaagtgtttttccagagattcctgcaggctggcctgggttttggagcacaactggctcacggcttcatgtttctttatcagaccagtcattgcacggcccaggctctccaactcagctgagtggtacttgcggcacaagctattgagattttcttgggtagagctgatgttgctttgttgactttgaagttctttttgtatatccttgacttttttcaatgcttcacaagtctcattttgggcacagttcatcaacgattcttccacttttgtgaaccatgttgttatgtcattaataaacttctccacttgtgtactttgagccgtgaaatccttcagggttccttttgctacttcagttatttctttggcatgctccagtttctgcattaagtctgcttctataaactgaaggtctggcggtgtttctagatttttagttaattctttcagatcattaactttggaatgcagttcttccaatctcaatgctttgtttttaacttcagactcaaattctttaagcagttcttcagctctgaggtggttatccaggttgctgatgttttctgccatctgtggaacgcagttgtttgaccatccctcaatctcatctctagttgacagtacatcatcccaaatggacaggcttactctcagcctatccatgttttcttcaagtttctctgatacatccagccatttgtccacggtgctctccatgtctgttttcaccaagctgaaatcactactgtgaattttcttcagctcagataacaagtgttttcctttgctggtaaagttatccaagtctttctgtttgtaattcattttgttcttggcagtttcatgcttggaaaaagcccatttaagatcctcctgatcttttatggtagttctggttacaatcacactgctggcattttctaagactttagatacagctgatttcaggttctgatattctctcattaagtcaataagtccacagcactgaccctgattttcatgaattagtcttttggtatcatcccaggtgacctctaagcggtttatctccctgtcaacttcaggtgcaaaagctacatctttctgggcaatttgcttggctttgtctttcaaccaacatagttcatgctcgtgagaattcaattcatcttctagctgattaaacactcttaacctctgctgaagagcttggcgggtaggttctttcaatcgctctttgtcagtcctttcttcaatgtcctcaatgcttttcagaagctcctctttctggtcttggaatgcttttttcaacactgccagagcatctgcctcactctgcttggttcccagaaggttctggatcctctctacctctccacagagctgatcagccgtggctctgcaggaagtcctttgctcagagctcccgattttcagatggtattgggctttggaaagaatgccatccagactgacggcagcagattctaatgctttagcattttgaagagcatcattgaggtccttttctatcaaatcagactcgttcttattcatactgttggttgcttccactgtttgcctcagctggcggagaatgccggacagagaggcatggctctggaggaattctgccaaatgggacagggcaagctgccgcctctccacaacctggctggcctcctcaaacagctggaagcagtcctcagcctttccctgcaggaggtggaggtcctcagcacggcccagagaacccaactttgctaagtgaccctgcagactctgcaattcgccctttttgctctctacttctgctgcgtggtccttatgccgagtaagggctacttgatggtccattatgctaatctcagaggtagtttgtaattcactgagaaacagtttaatccagacagaaaaggaaagcagcagctcatcaaattgctggtgttcagcaaccacagactgaagaaaattaatccttttgttaatgatctgtggtaaatctctccatctctcatccaactgctccaaatgtagtttcatcattttcacatcatctttggaggctactgagaacaatgattccttcaattgcaaaagtttgctatagaatgaggcctgggatacaacttcattttgcagtgcctgtattaactgaagttcaccttccactttgactctgtctgcagaaatgtccatttctggggaactggctttagcttcaccccgctctaaccaggtcaaaaaggatgatagttctttctctagcctctgccagtgggccagcagattctccagcgccgtctgtctctccttcgccctccttaggatgtcctcgtattgctgctgtagagccgcagcctcctgaacacaggaatctctgttcacaaccttcctggcactggctgagaaggcagtgatcgcgctgctcagtgactccagggcctggcagagatccatatgttcttgaagaactttgtatgtttctgtagctgaagaacatattttaattggaacagcaagtttatcttcaaattcagacacagattgctggatctttctaaggttctcttcaaacttttgctgctgagataaatgtcccaggattgttccttccagacactgtgcatgctctcgaagctcttccccgtatcttcttatttgtgtcaacttggctttaattcgagcagattctccagtggtaacaaactgagcaaaagactgggcttcttcttctaatcctacaatgctgctgagcttactttctatttcctgaattgtgaccttaatttggctgatttgcatgtccatggcagatgacgaagtttccaaggcattgagttctttttctttctcagttatccagacggacagagtctcaaaattactgccaaaatgatcccacttggttttcaccatttccatggttttaatatcttcttcaagcgtgtcttctaattttttgacttgttctttgattgacttggcctgctgttgaagcagctgcttattttggggcccaagcggtatctctgaagcttcctttacaaggttctcagcctggactgcaatactttctgtccgtttagaaaactcctttgtttgttccagttctgaagataaactttccaaactgctaaaactcaagaagcgttcatgactggaacctgtttgaaaaaggtatcttactactgtttctttgtttgtttcaaatcgctcccattttcttaatgtgacctggatgcggcgttcctgcctctcccggctgcgctccaggccatccagtgtgctctccagcttccgcagctcctcgtggcctcggtcaggcagccccccttctccctgctgcgcctgcgcgatctgctgctgcacatctctcttctttgctgagatccgctttgtcttttgctggtgatgaagaagtaactgctgtgcttcaaacagattttcagtatccaagatcttctcagcttgttcctggacttctttagagccagaaattaattcttcgagagaatttttgactatttctttgtactggacacagtccccaaaattgcttagcatcttttcaacctctgacagcagcgtcacaagagccttgaaagagctggataattttgccagctcatctccctgcttttgggcttcattctcagaagaaacttctgtcaaaactttcagcctggatttcagccagctgagggtctcaccccttttggtaacaccatttctgatctcttcaacggcacgtttaacctctccgtggttggcagtatcgatggcctcacccttgatcccctttaattgtgtctcatttgtagatatccaagatgagaactcagagaatctgctagtgtagtccttccacttgtctgggtcttccatgagcttcctgtaggtgctgtcaatggcagctctgagctctttgagagtcacgtgacaggttccaggtgtgtcccttactgggtcccgcactgggagtttcacacagagttcctcgatgagctgtaaccttttctcacagagatgatgaggacctttgtcactgaagaaaaccctgtgctctttaattatcttttcactgccttcctggggcatcagcttggtctctcgatccagctcagttctgcattcttctacagaggctaagaacctattcttctccacatcaatcttcagatgaagcaaatgataaggggcttctccttgaagatccttccattgtttgtggagctttcgaacagcttcctgcagcccctgctgctcctgctctggaaggatgtcggtgagttcatcacaagctttcaggaaagcattgagcaccctctgatccagctgactgaaaaactcagtgtgtctccgcaggagctcctctggatcccccttttcctccaggccctcctgagcaatccgcagtaccttctccaactctgctcgagactcctcaaacttcttcatcaagcgactgttggtttccacatgcttcttccaatctccagttttctttaccatactctgatgtttttgtttaaaaagggcactcgattgtgcctcacgctcaagaactgtgataatttcattgattttcccaagtgagtcataaaaggacgtcatctgcttttctaattcctccaacggaatcaacagctgctgagactcataaaggagtggggagtaacattctttgaccttggttagctgctctttgagctttgacatggtcgcaaacatttcttttccttcttcttgggggctttctttggtaatgaggtgtgctgtctttgtaattatcttgtattgggcatccatcacaggcaccctctgctcaatatcctccaagtcttgaattaatagcttgacattcataaaagagacttctaagggttcagaaagtttcttatgggcttccgttgcaaaagcagacagggtaacaacacagtctgtgtattccttcttcattctgtccatctcatcagcttgagcatattgcttgacttccataaacaactccctccaccgcccatttagcaacagtaattgctgcttcaggtcacgggaaaccatctcatcacaggtttcaattagaaaattgccagcatcgttcatggcagtatgctgctgaatccaatgaggtaaatttcgaaaaaaatcctttttggcattttctgattgattgagcattttttcagcatcctctagccaggcttgcagactagccactgtattgccatagcgatcccagttagagatcacttcttccagcatgctcctcacactcctcacttctactgagagattcctccactgagcggtggtttcattcatgaatttcatcacattctcagcttcttccactgaaccatctgctttgacatacatctcagctgtctgtttcaagatctggtatgtcacctcatattgttcaaagaacttgctattttctataaaagacacgtagttttgtagaagctgctccactgactctctcctcccgtacttaatgatccaagacttcagctttgactctgcaagaaccagcagtgagagcagacggtactttaattctaaaaattccattttcattaggtgtagctctgatgtggaggaaacaaaatgaaacctctcggccatgtcctctaattgatcaggtggcactggaatcccgttaacagacctggtccggtagatttcatggaatgctcttttgtgggcatccgtgttttgaagcagatccttatgttgctcaagtttccgttgtatcgtgtttgctgtttcctcgtggacctgttgaacggttatttcctctctcagggccacctccgctctgtacagccaggcacctatggtgcccagaggtgcaggaagagatttatcaagctgtatatgccagtcaaagagcctggaggtcactctatcccaagattgttttaccaatgcttggtcaagtgacaatttaccgtctctgtgtaatggttgtattaaatgttcaatctgtttcctcttcatttcatattgaactctgaagtgcttaaatgactgatatttatcctgtaaatttgattccaccatctgtgctcttgtcaaatctctctcaaattgttctatccaaactttcatttccttaaaaattactctgtcttctctcttaaaattttgtacagaatttgcaaaagatgggaaacctggaagtatttcatcatcctcttgcccatcagtgcttgcattgtggatgtcaggataatgtttcagaaactgggctacataggtcataatagatttctcatctggtttatccacatcaacgtcttcaggatctagcagtcttgggatccccagttctgtttcggcgatagtgaaagcatcctccaaattttctcggttggatctgcctttcactgtctccaagtccaccaattccggtcgaatggcatgaataactgaatgaaaggcaaccccgcttctccaactcttcccaaaatcttttacttctattccagtctgcttgccagctgtgtactgaacccactttaataaagccttcttagcatttccttggatcttggtggtcaccttccgtttacttggtgggctgggagtctcagagctaactatgctgtccacggaggatgcgctgctggacaaagactggagctggggcaggttgctggtcaactcttcaatctggaaatatagaataatggtccacatcaatccaagaactattgagggtcggccatcagctatatcggtggagttaatgttgactaatttaatcggtgatcctctgtgcatggactttcttccttcgaggaacttgagtgccgtgccaatgttagccacagcatggattcgcttcatccggcgtccttgttcacaaggcagtttctgcccagacaggacctccagaagggcaagcagtttaacaccatctttcatgtcttcaaaaagatcgtccaccaccattggaggtttccgcttggccagatgagagttgatccattttgtgaaagttcgtttttgtactatctcttgctcatcttgcagcctctgcatcacattggcgatatcccgaggacaccgggaggcccctctggaggttgccatggtccctccggaagcacgaagccaacaccaagagactcttcactggaggcagcacagggctacaccactctagaaaacatgcttggacttttctagatctattctgtcataaatgaattccaggcctttgcagcactcaacaaggaggcagctctcccaaagactgaactgcttctttttcttcttccgttttaagactgtcctcttacatgaactcaagaaccttctctctcggcctcgttcagtttcccagcagcaaggcgaagcgagcgaacgcttcctcccggctctctgcgcccaggctcggcgggaccccggggatgcgcggctgtccgcccgccctgtcgccgggatcgggcgcggtctgcaggactgcgggagcccagccgccctggtgacagaggacaacaatctcagcccgctgcggccggcggccgcggcccggcgcccgcgctcaccctggctggctcgcccacact

SEQ ID NO: 9581 - RNA, 13961 nt, Homo sapiens
  source 1..13961: mol_type = other RNA
agttcttcagtggcaagctttatcaaaatcttccttaaaatgcttcctagaaaccaaattcttctctagttcttgtaaccggtgactgcacttttgtaaaacactgtcatagacactctgcaattcctgaagcttccccagcacttcactcttttcctgctctgtgacttccttcattagttcgcgaccctgggcccaaagtccagtgacttcattttggtaagtcttgaggctggcttgtgcactcttacatgttttgacttgtttgctcacatcatctggtaacagacagatgtgttcacggaacattatctttcgctcatgttgctgaatttggctggtggcctggaacactgccatgagaaactgggttttctcggacaaggctttgtttaagtactttcttcgctggcccactaagtcactgagacaattcacgtggctttgtgcatcagagagagccttctggatgacctgtcgctcattgagaccaagatctgccatgaccctgtctgcgtcctttataagcgatttcaggagcatctgcttggcctccagttcactgcagatggccaggtgatccatgagaaggttctgagccatatctggaggagggctctgcttaagggcctcggcgatgttgggttgttgctcttctgcccactccattagctcctgaaatctggactgcaccacatttaactcctccaagttggtgactgacacttggattttccttttaatgaggtcctcaagctgaaaccaacgttgctctaaatgactcgtctgttctttgactaactccttgtcatctaaattcagatgctctatcattttctgcttttgatctttcagatcttcaatagcatactttctctcctgcaatgccaatgctaactttttcaaagcttccaggtggacagctgtactctctgcatcagatctggccaagttatcccattctgtagtaaatttttctaggaacacttcaacaacattcatacagtcatggtaatctcttgttctctgaagatcctcttccctttgcaagcacaggttgttagactgacggcacaaatcgagccactgatcatttaaatgatttatttccttgtgttcaggcgattcctccttctttgttaacttattcaccttttctattatggtgttcacggatgcctgtttgctctgtagtttcttaacaaaatccttaacttgtgaaaccatgttctgtgcaatgttcagctccagctcagagtgcctcctcttcatgttctgcagttgctgatcagcatcttgcaggtaaatccagagctcagacttcaggtgcttgatctcttcccagccctgagttaagttctgggcctggacaagcttttgttcaatcgtttgctctgtttgttgaatgtcttttgctgtggttttcaccgaagcatttgacaggtcacacatggagcaaaggagatctaggtaggtccttgcctgctcttgcaaagctctgaagtgtttgacctgcttaatggcttctgccctactaagaggtggttgaggacttggctctaaatccggctggactgcagaaagccaggcctggcactgctgcagggtgtcttgtcggctgacgtgcttctgaagttcgtgttccaaactctggtacatcctctgagctgtgctgcagatcgctgagtagctgtcctttgtgccctgcagatgagcatgcacgttttgtttaagtttcgcttgcaggtggtctgcacattggccaatcaaagtatcacctttcatttgaagattgttcaaacggtcttcaaaaccagcaatttcttccatcattgcctttcctatgctgcacaggtcctggtaatcactttgaagttgatctattttgtcctttaaagtgacgtcctgcaccagttccaaaagagcttcacccttctctctcactgactttactgatggttcatgggacagcaccgtttgttgaagtgacttgtatttagataactgagcttttttctcatataattccattttgggttcttcaggaacatgtagaatttcctggtattctgctatccactgtgtcagtgctttgcatttatctgagaattcctttgctaaatgaagacctttttccagcgtcatgtgttctttccggacagtgctggtcagttccttcaactgctccatgtgatcatgaatctcctttcttaacctctctgcctcgccttcctccaagtatttaacagccctctctcctttctcccgggctgatttcagcaaactgtgacctttctccatgtctttgagcaaaacctccaacgtcttcaatttcttccccatcattactgtatctactttgtcaatcttggtagccacattcttgaagtttttatgagtagagccataccaatcagaataggaactgagggatgattctgattcctccaaactctgaatctcctcctccaggaattttatttgttccagcacttggagaagcagggcctggtatctggaagtcagctgggtggcctggcaacccattctgctgttcacgtggctctcgtccagtatctcctgagctctagctcccacttcctcaacttcatctctgtatgcagtcacttcttcgtgccactttttctcctctgctgttttgagccattcatctacttgctgaaacttttgctccattagcctcaatttgttcaccacgttattgaactgagttcgagtctcggacagcctgtgctggtaagcctgccagtcttgccggagagactctaaagcccggtcctctgcctgtgggatacctgatgggatcacatcctctctggtgtgcagcactgagttcaacagggcctgcccctctgcacagtgtacctgtagctcctgaagatcacgcaatgttgtctcatgagtgtgggcatcaccttcaagaactgaatactggtcgagcttttcttgttcttgccccaaccaaacttcaaatgcctttaggtctctctgatactcttggtgcaggcggacaagtttttcagacttggttacggcttccttggccctctcttggatggctctgtatcgttcctgtagatcctggagttctagctgggtgacatagtgttctgtcatgccagcccctttgacttcgatggtctccagcaagctgctgtaactcagcacttcttcatttaataacttggcttttccgagcatcgttgttttatcccgcagctccgcatgctgcctttctgattcattcaggttggcttccatactatccatccaaccggagaactgtcgaacgccatcctgataacttgtccacttggagagagctccttcgagttggcttttacaacgaatccctgcagacaaaagggatgcccacatatccttcacactctgcagctgctgctgaatagtgggaatgccttctggagaagtattctgaaggacagattctcccctggtcactatcattttcatctgaatctctttttcctgtttgactgataatagagcctcgagcttgagcgtcctgctgtccagcacacttttgtcggatgtcgggtggcagtatgaatccagcatgtgaatcgcatccgtcatccagtcttgtaattctttaatcccaagagagaactgattgtgttctgcaacgattctatccagtcttgacactttctcctttgttaaattgcttagcgctagatactgagaagacagctgcgacactctgtgcctaaagctcttgctggcagcttgtccttcccacagctgctgagctttctctttcagcctgttgagctgaggctcgtagcagtgtatttcctcaaggacagactggagcttctgctgctccctcctctttgctggcagatcatagaggcgattgctgctttcatggaccatcttctcagttttactcagccagtcctggataggctcagcacttacttcaaagtccttcatttggatctttagattctctagagcagattctttttggtggagatttgaatgaaaatttttccaatcttcttttgcagctgtaactttggcctggatccctttcgctttctctttggtcagcagggtactcagaagttcccctttagacagcatcatgtttagcttgtgctgtccattttcactttctgacaaaaactcctgtattttctgaagactagttgaaacttcacttatattttgaggtatatcaaaacacttggcggtagtgatttttgcattaaccaaccactgctggaaatccctgaaggcctttcgaaatctttgctgtaaaatctgttctttattctggcagcccttggatgcttgcaaacaaagacaattatactctttaatcaagccagaaacttttccactgtaggtactcaggtctctggaaaatcgacaaagttcattcagctgagacttgagatcctctgttctaggctctgctttttgcaaagcatccagtatctcttgtcctttgtgccagcattccactatctcctcatccgtgttcttgccttccaggagggttaactgctgagcccaggttttcagaagggcactgaactgttccagggcctgctccagttgagccacttggcctgagaattcctgctccgaaagggccatctggctgaccaggttctccaaacagctctgcgtttggaatacactgtcttcccactgcttccagtcggcacgcagggcctgcatctccgtgtgcatgagctcacacccactggcagttgtgttctgtttcacttcgggagccagcgactccactctgctgagacggcttgcaccaatctctctggaatctatcagctccttaatttttgataactttttctgggtggctgatgaatctccagacatatctgaccaccggtgaagttcttcctttgctgaatggagccaatctgtgaactcgtggaccgcatctaaatacattagatgatctttcacaatctcttccactttcctcattttttccttggcaacagtcattatatcattaaactgtgttttcagctcctcttgagctgtgtccttgaaagactcatcctctgtcttttcgtagagctccctggacttcgcaattagacggtgaagggctctcgtgtgatcttctgcctcagacaggatggactggaggtggtcaagcaggacgaacttctctttcagacctggctgtggttgtaagggatgttctattttttgatccactgattccatccactgctccaactggtttttcctctctacatagtcattccattggctaatcacagactctaaagtgctttgagcgtggacggaggagctcatgatgtcagcccacacttctttaagggtctctaactgagtctgaatcaccctctgaccttctttgttgctacttctcaaggcctgttcccccttgccaatggccatattcaacttaacttccccttcacctttcatcaggagaatatcctgtatttgtgacagccgtttctccagggtgtctttgctcccaagagtgctctctgcacaggccagtctgtcctgaatggccttcacccagaaccacatgctttgcagtgcttcctccagggcttcgtgctcctgaagggccacctggcagctccggagtttctctttggtcattctaagtaggttctggtggcttgtgaggagctgggaacacaggcggccctcctgcccagcaccgtggccttcttcactcagaagctgccctctctgggaaagcttatcaagagactctcttgcagccagcagttctcccaaaaacatttcaactttatgaacttcatttttcttctcaggaatgtgctgtttactctctcccaagttttccgtattgaacctttcttccatttcatggatccataagttcagttttctgtgctgatcttcaaagcttccaagttctgaagcacagtcttgaagagcctgcttatctttaaggcattgtttcagaaatgcttgaaactcttcattggcctttgtgatttgttcttgaatgctactgacaatttgtttagacaaatgtgcatacaaagtttgtccttcttgagtcactgcatcaagtttgctctgcccatcactgactgagtccaaaatgttctgaagatcatggagctttgcttctagaactttgctgtcaccggtgcgatctgatgattcttttgctgctgcctttgctcccaaaaaccattcttggaattcctgcatagactcactgaagtgtttttccagagattcctgcaggctggcctgggttttggagcacaactggctcacggcttcatgtttctttatcagaccagtcattgcacggcccaggctctccaactcagctgagtggtacttgcggcacaagctattgagattttcttgggtagagctgatgttgctttgttgactttgaagttctttttgtatatccttgacttttttcaatgcttcacaagtctcattttgggcacagttcatcaacgattcttccacttttgtgaaccatgttgttatgtcattaataaacttctccacttgtgtactttgagccgtgaaatccttcagggttccttttgctacttcagttatttctttggcatgctccagtttctgcattaagtctgcttctataaactgaaggtctggcggtgtttctagatttttagttaattctttcagatcattaactttggaatgcagttcttccaatctcaatgctttgtttttaacttcagactcaaattctttaagcagttcttcagctctgaggtggttatccaggttgctgatgttttctgccatctgtggaacgcagttgtttgaccatccctcaatctcatctctagttgacagtacatcatcccaaatggacaggcttactctcagcctatccatgttttcttcaagtttctctgatacatccagccatttgtccacggtgctctccatgtctgttttcaccaagctgaaatcactactgtgaattttcttcagctcagataacaagtgttttcctttgctggtaaagttatccaagtctttctgtttgtaattcattttgttcttggcagtttcatgcttggaaaaagcccatttaagatcctcctgatcttttatggtagttctggttacaatcacactgctggcattttctaagactttagatacagctgatttcaggttctgatattctctcattaagtcaataagtccacagcactgaccctgattttcatgaattagtcttttggtatcatcccaggtgacctctaagcggtttatctccctgtcaacttcaggtgcaaaagctacatctttctgggcaatttgcttggctttgtctttcaaccaacatagttcatgctcgtgagaattcaattcatcttctagctgattaaacactcttaacctctgctgaagagcttggcgggtaggttctttcaatcgctctttgtcagtcctttcttcaatgtcctcaatgcttttcagaagctcctctttctggtcttggaatgcttttttcaacactgccagagcatctgcctcactctgcttggttcccagaaggttctggatcctctctacctctccacagagctgatcagccgtggctctgcaggaagtcctttgctcagagctcccgattttcagatggtattgggctttggaaagaatgccatccagactgacggcagcagattctaatgctttagcattttgaagagcatcattgaggtccttttctatcaaatcagactcgttcttattcatactgttggttgcttccactgtttgcctcagctggcggagaatgccggacagagaggcatggctctggaggaattctgccaaatgggacagggcaagctgccgcctctccacaacctggctggcctcctcaaacagctggaagcagtcctcagcctttccctgcaggaggtggaggtcctcagcacggcccagagaacccaactttgctaagtgaccctgcagactctgcaattcgccctttttgctctctacttctgctgcgtggtccttatgccgagtaagggctacttgatggtccattatgctaatctcagaggtagtttgtaattcactgagaaacagtttaatccagacagaaaaggaaagcagcagctcatcaaattgctggtgttcagcaaccacagactgaagaaaattaatccttttgttaatgatctgtggtaaatctctccatctctcatccaactgctccaaatgtagtttcatcattttcacatcatctttggaggctactgagaacaatgattccttcaattgcaaaagtttgctatagaatgaggcctgggatacaacttcattttgcagtgcctgtattaactgaagttcaccttccactttgactctgtctgcagaaatgtccatttctggggaactggctttagcttcaccccgctctaaccaggtcaaaaaggatgatagttctttctctagcctctgccagtgggccagcagattctccagcgccgtctgtctctccttcgccctccttaggatgtcctcgtattgctgctgtagagccgcagcctcctgaacacaggaatctctgttcacaaccttcctggcactggctgagaaggcagtgatcgcgctgctcagtgactccagggcctggcagagatccatatgttcttgaagaactttgtatgtttctgtagctgaagaacatattttaattggaacagcaagtttatcttcaaattcagacacagattgctggatctttctaaggttctcttcaaacttttgctgctgagataaatgtcccaggattgttccttccagacactgtgcatgctctcgaagctcttccccgtatcttcttatttgtgtcaacttggctttaattcgagcagattctccagtggtaacaaactgagcaaaagactgggcttcttcttctaatcctacaatgctgctgagcttactttctatttcctgaattgtgaccttaatttggctgatttgcatgtccatggcagatgacgaagtttccaaggcattgagttctttttctttctcagttatccagacggacagagtctcaaaattactgccaaaatgatcccacttggttttcaccatttccatggttttaatatcttcttcaagcgtgtcttctaattttttgacttgttctttgattgacttggcctgctgttgaagcagctgcttattttggggcccaagcggtatctctgaagcttcctttacaaggttctcagcctggactgcaatactttctgtccgtttagaaaactcctttgtttgttccagttctgaagataaactttccaaactgctaaaactcaagaagcgttcatgactggaacctgtttgaaaaaggtatcttactactgtttctttgtttgtttcaaatcgctcccattttcttaatgtgacctggatgcggcgttcctgcctctcccggctgcgctccaggccatccagtgtgctctccagcttccgcagctcctcgtggcctcggtcaggcagccccccttctccctgctgcgcctgcgcgatctgctgctgcacatctctcttctttgctgagatccgctttgtcttttgctggtgatgaagaagtaactgctgtgcttcaaacagattttcagtatccaagatcttctcagcttgttcctggacttctttagagccagaaattaattcttcgagagaatttttgactatttctttgtactggacacagtccccaaaattgcttagcatcttttcaacctctgacagcagcgtcacaagagccttgaaagagctggataattttgccagctcatctccctgcttttgggcttcattctcagaagaaacttctgtcaaaactttcagcctggatttcagccagctgagggtctcaccccttttggtaacaccatttctgatctcttcaacggcacgtttaacctctccgtggttggcagtatcgatggcctcacccttgatcccctttaattgtgtctcatttgtagatatccaagatgagaactcagagaatctgctagtgtagtccttccacttgtctgggtcttccatgagcttcctgtaggtgctgtcaatggcagctctgagctctttgagagtcacgtgacaggttccaggtgtgtcccttactgggtcccgcactgggagtttcacacagagttcctcgatgagctgtaaccttttctcacagagatgatgaggacctttgtcactgaagaaaaccctgtgctctttaattatcttttcactgccttcctggggcatcagcttggtctctcgatccagctcagttctgcattcttctacagaggctaagaacctattcttctccacatcaatcttcagatgaagcaaatgataaggggcttctccttgaagatccttccattgtttgtggagctttcgaacagcttcctgcagcccctgctgctcctgctctggaaggatgtcggtgagttcatcacaagctttcaggaaagcattgagcaccctctgatccagctgactgaaaaactcagtgtgtctccgcaggagctcctctggatcccccttttcctccaggccctcctgagcaatccgcagtaccttctccaactctgctcgagactcctcaaacttcttcatcaagcgactgttggtttccacatgcttcttccaatctccagttttctttaccatactctgaaaagcaacatgaatatctgcaatctgtctttgtagcctcgtctgatcaaaatgctttaacacgttgctcaaggtcacaaacttttgaacactttgactgcctttctcaataagtgtcaaggttttcttacagttttcttgacaagctaacagttcctgatgtttttgtttaaaaagggcactcgattgtgcctcacgctcaagaactgtgataatttcattgattttcccaagtgagtcataaaaggacgtcatctgcttttctaattcctccaacggaatcaacagctgctgagactcataaaggagtggggagtaacattctttgaccttggttagctgctctttgagctttgacatggtcgcaaacatttcttttccttcttcttgggggctttctttggtaatgaggtgtgctgtctttgtaattatcttgtattgggcatccatcacaggcaccctctgctcaatatcctccaagtcttgaattaatagcttgacattcataaaagagacttctaagggttcagaaagtttcttatgggcttccgttgcaaaagcagacagggtaacaacacagtctgtgtattccttcttcattctgtccatctcatcagcttgagcatattgcttgacttccataaacaactccctccaccgcccatttagcaacagtaattgctgcttcaggtcacgggaaaccatctcatcacaggtttcaattagaaaattgccagcatcgttcatggcagtatgctgctgaatccaatgaggtaaatttcgaaaaaaatcctttttggcattttctgattgattgagcattttttcagcatcctctagccaggcttgcagactagccactgtattgccatagcgatcccagttagagatcacttcttccagcatgctcctcacactcctcacttctactgagagattcctccactgagcggtggtttcattcatgaatttcatcacattctcagcttcttccactgaaccatctgctttgacatacatctcagctgtctgtttcaagatctggtatgtcacctcatattgttcaaagaacttgctattttctataaaagacacgtagttttgtagaagctgctccactgactctctcctcccgtacttaatgatccaagacttcagctttgactctgcaagaaccagcagtgagagcagacggtactttaattctaaaaattccattttcattaggtgtagctctgatgtggaggaaacaaaatgaaacctctcggccatgtcctctaattgatcaggtggcactggaatcccgttaacagacctggtccggtagatttcatggaatgctcttttgtgggcatccgtgttttgaagcagatccttatgttgctcaagtttccgttgtatcgtgtttgctgtttcctcgtggacctgttgaacggttatttcctctctcagggccacctccgctctgtacagccaggcacctatggtgcccagaggtgcaggaagagatttatcaagctgtatatgccagtcaaagagcctggaggtcactctatcccaagattgttttaccaatgcttggtcaagtgacaatttaccgtctctgtgtaatggttgtattaaatgttcaatctgtttcctcttcatttcatattgaactctgaagtgcttaaatgactgatatttatcctgtaaatttgattccaccatctgtgctcttgtcaaatctctctcaaattgttctatccaaactttcatttccttaaaaattactctgtcttctctcttaaaattttgtacagaatttgcaaaagatgggaaacctggaagtatttcatcatcctcttgcccatcagtgcttgcattgtggatgtcaggataatgtttcagaaactgggctacataggtcataatagatttctcatctggtttatccacatcaacgtcttcaggatctagcagtcttgggatccccagttctgtttcggcgatagtgaaagcatcctccaaattttctcggttggatctgcctttcactgtctccaagtccaccaattccggtcgaatggcatgaataactgaatgaaaggcaaccccgcttctccaactcttcccaaaatcttttacttctattccagtctgcttgccagctgtgtactgaacccactttaataaagccttcttagcatttccttggatcttggtggtcaccttccgtttacttggtgggctgggagtctcagagctaactatgctgtccacggaggatgcgctgctggacaaagactggagctggggcaggttgctggtcaactcttcaatctggaaatatagaataatggtccacatcaatccaagaactattgagggtcggccatcagctatatcggtggagttaatgttgactaatttaatcggtgatcctctgtgcatggactttcttccttcgaggaacttgagtgccgtgccaatgttagccacagcatggattcgcttcatccggcgtccttgttcacaaggcagtttctgcccagacaggacctccagaagggcaagcagtttaacaccatctttcatgtcttcaaaaagatcgtccaccaccattggaggtttccgcttggccagatgagagttgatccattttgtgaaagttcgtttttgtactatctcttgctcatcttgcagcctctgcatcacattggcgatatcccgaggacaccgggaggcccctctggaggttgccatggtccctccggaagcacgaagccaacaccaagagactcttcactggaggcagcacagggctacaccactctagaaaacatgcttggacttttctagatctattctgtcataaatgaattccaggcctttgcagcactcaacaaggaggcagctctcccaaagactgaactgcttctttttcttcttccgttttaagactgtcctcttacatgaactcaagaaccttctctctcggcctcgttcagtttcccagcagcaaggcgaagcgagcgaacgcttcctcccggctctctgcgcccaggctcggcgggaccccggggatgcgcggctgtccgcccgccctgtcgccgggatcgggcgcggtctgcaggactgcgggagcccagccgccctggtgacagaggacaacaatctcagcccgctgcggccggcggccg

SEQ ID NO: 9582 - RNA, 3109 nt, Homo sapiens
  source 1..3109: mol_type = other RNA
agttgccagggctgcctttggtctcacactcatcctcatccccatcagtggggacacacactccaaagcacagtgatccatgtgcatgggagcactcccaccctcctcttgccctgtggacctccttgttcaaaactgtcctctgctcagactcaggccaggaccccagctttttgcttcctggatccaaaaggggggacccctgcacctctgctggggggcatccatcatattcattgatgatttttttctcaagtattccataaaatcccttgccgggctgtggagacagggctgcgttgctcctgagcgcctcacctccacccctacctgcctctcctgcggggcccactgctctgtgctccgtggaagggcccactgtccctggcctgctactgccctggcccttccttcagtgattaatgctcctacaggacgccttgggaagcctccatagcaccaagcctgctcttgtcacaagagaggagcacagtgcagacacagtgtctactccctggaaggcagggccatgtcctggtggtcagacccaccaggtggattgaacagaacagagcatagtcccgaggatctgcatgggccttcctatgggcagggcatctgaagagggagcatctcgtttcttcctctccacagccctggagggaggcgagggggaagggagcagcagggctattgggggatgggcacgggcagccctgggtcccaggctgggatgtgtctgcacattggcaccactccctcaaccagggcgctttctccctggaagtgtgggtaacagtgtacaccccagaacaggcagagggagtgctcttgatactctatacttcacacttctatgggtttcttagtctccacatcttgtaaacaaaggaaactaggtctgcacaatccccaacatcatcacagaaacagattctaaagctggaaggaatcagagatgatgaggtccactccccctcattttacagaaggaaaacctggtccccagggcaagagtgatttgctgaatgtcatcaaggcaatgggaggcgttcctgccttggggccacactcctgctgctccagaaccccagtatagaatagcaatagcaggatgcctggtgcaatgaacaccagacaggtggagaagatggcttcagcaaggaagtagaaatggaagaaaagccaatttctggccacagctgggaaggcgatgtactagggcagaacaagagggtctccaggcatggacaaatggctgctgtatttctaagaacagaagcctttttctgttgctaggggcgagagctccttttgggcaagctcttacatggaataaaaagggtagaattagggcttgatgtgggctgggcggtgagaagcaggcggggggtggtggtgtggctgagagaagagcctgaagggaggctcaggttctggctcaggctccagaaggtggtccctggccctgaagaatgactgagcagagccattggggggccccaaagccccgtgctcagctctaggctgggcagggtttgcagggagtgtccatctcaaggctctgcccagctgtgggggtggcattgaatcagcacagatcttgggccgaagcacctgggacgttcccaggaggccccaagggccccacaaacccctcagaggggaggggagggagcatacttgctccagaacttggagcctcttggctgaaggggctggaggagaggagcccctggtacaggctttcaagtgaggggaggggctggagaggggaaggaaagtgatgtgggaggaggggtgggggcagcattctgggaaggtgtccccacgcaagggagtggagggacagacacgcatggccatgttcttgctccaggcctgggaccctctcctcaccttccaactcaactcctgcagtttcagccgtcctccacagaggagaggctgcctagtgaaggcctgagttggccagcagcagcacagaagttccactggcccgtccaccctcacccacaccccatactgggggaagcgcagttccccagggccatctcaccagctagcccggcactactgggaggtgcagacaacctgccagtatccccattttgaatagacagcagaagtatttggggctcacacccacaactgctgccactgatgcagtggggggctcatccaacagagagctggccctcgcccgtgagcactagggagtcaggtccctctccccagcagaaggatatgaggacattctctatggagcacctgcttgctgctctgggccacctgccaggccctctgcccctaccccaaactcctcctcttgcactgtcccaggggtccctccaacccaggccttgatgagtggggagctctgtccctagcaggaccccctggccatcctgcagctttctccctgcacagggaagcacaggtaggagccgagggccacgtccaagagctgctcagctgccagcccttctcagcttcccgcgactcccacctccaggtagtttctttctcaggccggttctaacacagagaaacacgctggcaggcctgcggctcctcctgagccccgcagctggccacagcccacctgccctctgttctctctccctcccactgtcccactgtggcctccctacccctctccttcctctcccctctccctttccctctgctgcgggagagcagcacaacctttgcattccaggctgcatgcaggctcattcatcccacggtccctcttcaagctatggggcttctgcaggaattcctgttgggtctttgagcccacaggccctcctcgctggtagctgcacagagtagaaatgctggcctggtaggaaggatgggaggagacctgcatggggccctgggctcacgccagctcttcctgcgggtttctggtctggtcagagagctgcaggtgggagtcactcttggagaggcccagaccccatctgcaccagctgggcagccctgaagccaaccttcctctctggagatggtctctctggacccgaggtccaagctcagcccagggagcgctctgaagcctaggcctattcagatcctccccagccagtggaccttggcc

SEQ ID NO: 9583 - RNA, 6491 nt, Homo sapiens
  source 1..6491: mol_type = other RNA
agttgccagggctgcctttggtctcacactcatcctcatccccatcagtggggacacacactccaaagcacagtgatccatgtgcatgggagcactcccaccctcctcttgccctgtggacctccttgttcaaaactgtcctctgctcagactcaggccaggaccccagctttttgcttcctggatccaaaaggggggacccctgcacctctgctggggggcatccatcatattcattgatgatttttttctcaagtattccataaaatcccttgccgggctgtggagacagggctgcgttgctcctgagcgcctcacctccacccctacctgcctctcctgcggggcccactgctctgtgctccgtggaagggcccactgtccctggcctgctactgccctggcccttccttcagtgattaatgctcctacaggacgccttgggaagcctccatagcaccaagcctgctcttgtcacaagagaggagcacagtgcagacacagtgtctactccctggaaggcagggccatgtcctggtggtcagacccaccaggtggattgaacagaacagagcatagtcccgaggatctgcatgggccttcctatgggcagggcatctgaagagggagcatctcgtttcttcctctccacagccctggagggaggcgagggggaagggagcagcagggctattgggggatgggcacgggcagccctgggtcccaggctgggatgtgtctgcacattggcaccactccctcaaccagggcgctttctccctggaagtgtgggtaacagtgtacaccccagaacaggcagagggagtgctcttgatactctatacttcacacttctatgggtttcttagtctccacatcttgtaaacaaaggaaactaggtctgcacaatccccaacatcatcacagaaacagattctaaagctggaaggaatcagagatgatgaggtccactccccctcattttacagaaggaaaacctggtccccagggcaagagtgatttgctgaatgtcatcaaggcaatgggaggcgttcctgccttggggccacactcctgctgctccagaaccccagtatagaatagcaatagcaggatgcctggtgcaatgaacaccagacaggtggagaagatggcttcagcaaggaagtagaaatggaagaaaagccaatttctggccacagctgggaaggcgatgtactagggcagaacaagagggtctccaggcatggacaaatggctgctgtatttctaagaacagaagcctttttctgttgctaggggcgagagctccttttgggcaagctcttacatggaataaaaagggtagaattagggcttgatgtgggctgggcggtgagaagcaggcggggggtggtggtgtggctgagagaagagcctgaagggaggctcaggttctggctcaggctccagaaggtggtccctggccctgaagaatgactgagcagagccattggggggccccaaagccccgtgctcagctctaggctgggcagggtttgcagggagtgtccatctcaaggctctgcccagctgtgggggtggcattgaatcagcacagatcttgggccgaagcacctgggacgttcccaggaggccccaagggccccacaaacccctcagaggggaggggagggagcatacttgctccagaacttggagcctcttggctgaaggggctggaggagaggagcccctggtacaggctttcaagtgaggggaggggctggagaggggaaggaaagtgatgtgggaggaggggtgggggcagcattctgggaaggtgtccccacgcaagggagtggagggacagacacgcatggccatgttcttgctccaggcctgggaccctctcctcaccttccaactcaactcctgcagtttcagccgtcctccacagaggagaggctgcctagtgaaggcctgagttggccagcagcagcacagaagttccactggcccgtccaccctcacccacaccccatactgggggaagcgcagttccccagggccatctcaccagctagcccggcactactgggaggtgcagacaacctgccagtatccccattttgaatagacagcagaagtatttggggctcacacccacaactgctgccactgatgcagtggggggctcatccaacagagagctggccctcgcccgtgagcactagggagtcaggtccctctccccagcagaaggatatgaggacattctctatggagcacctgcttgctgctctgggccacctgccaggccctctgcccctaccccaaactcctcctcttgcactgtcccaggggtccctccaacccaggccttgatgagtggggagctctgtccctagcaggaccccctggccatcctgcagctttctccctgcacagggaagcacaggtaggagccgagggccacgtccaagagctgctcagctgccagcccttctcagcttcccgcgactcccacctccaggtagtttctttctcaggccggttctaacacagagaaacacgctggcaggcctgcggctcctcctgagccccgcagctggccacagcccacctgccctctgttctctctccctcccactgtcccactgtggcctccctacccctctccttcctctcccctctccctttccctctgctgcgggagagcagcacaacctttgcattccaggctgcatgcaggctcattcatcccacggtccctcttcaagctatggggcttctgcaggaattcctgttgggtctttgagcccacaggccctcctcgctggtagctgcacagagtagaaatgctggcctggtaggaaggatgggaggagacctggaacaggagtgaagcagatgaggttgaaataatgcaaccgttagaagaaacttcttgagtaaatttggagattaaaaacattctccagcatagccaatgtactcactcgaaccctggatggcagagattaatgaactatgggatggaaagttaacctccaaagatctcgctcaggaataatataaatttgttgtcctgggtatagtaatcaaatggacagctagcgctatagtacaaatacttgtatcttttctttggcggaaggaacaacatttgaaaaaaaggagcttatacatttccctcttttctcttcatacataaagaaaaaagcatttgatgcctttgttaggccttttaaagcaatgcgcacagggcaggaccatcccatcccccgctgctttaatcaattctgtgtctgctctccttgtttgactccaatcttaaatcttcgggcatcttcaggaaaaattcccacaaagggatccaggagatcatcccatccacccactacctggattggcctcccagccccatccccagcaaaggagcagtcatcttgtgctcaaaagattcatttacccctaatcctctcctcacccagactgctggacgcctgtcttgggctaggaggacaggctcttcatccacttattcactcattcattcatttgtccatcccacagtgcagaactgggaggcacccagcgttcagcacattagcactgaggagccatgggttctggacattcccagagtcccaattgaataaaatttcattgttttaaagtgaaggttgatgtttcaataaatcctttaacgggattttaagcctttctgtgagtgaatccacagtctacacgttctgatttctgcttctgctgcatggtagctaaggaagagcctgtggctgtgtgaatggaaaggcaccgatggctcatggtcatgggtggtgccagctgggatccccacaggaatcagccttggtaaaggggaacctaaatggctggcagctcagaagaacctgggcctaggggcattgtccaatggctgtagcctcatgagagaccaatttctaaactcaaaataccaactatgtcttgtttattatttttattttttgagacagagtttcactctgtgacccaggctgcagtgcagtggtgtaatcatagctcactgcagcttgtattttttgtggagatagggtctcctgtgtttcccaggctggttttgaactcctggcctcaagtgatcccccaactgcagcctgggattacatgtgtgagccaccatgcacggccccagttatttacttaccctgagaaatataactgtcatggggaccagaaccctcatcagtgcattctccctgtagattatggatgggggaaggcgaatcctaagtggaagctcagggcagaagtcagattggacagagaggtgtttggagttgcacttgtatagctcttcattgagaagaatgttgacattaaacacaacagctgtggaggatctttggcaaccaggcagagagaggcctgtggccacagtgggactgtctgcccttctttctgactccaagcagctgaaatcttcttatgtgtggggacgcttccccacgctctattaaacagaaagcctgcctccttttacagaaatgcaaaatcccagacactcactttttcttttttcttttcttttcctttttttttttttttttgagacagagtctctctctgtcactcaggctggagtgcagtggcgcgatctcggctcactgcaatctctgccgcccaggttcaagcgattcttctgcctcagcctcccgagtagctgggattacaggcacctgtcaccacgcctggctaatttttgtagttttttagtagttacgggatttcaccatcttggccaggctggtcttgaactcctgacctcgtgatccacccacctcggcctcccaaagtgctgggattacaggcatgagccaccgcgcccatcctgtactcactttttcatactcctttgcaggttggctgtgataggtgtccctggccacgtcagtggagcacccaggcctcaagcagcatgctggggaagggaaaaccccccattctggtgatggaggtggccatgaccatgtctggttttcaaaggcagctttgtaagaacagaaaccagcagctccccaacatctggccctatctgctgtgcaaaccacagggaccaggacctttccggggtgccagtggcatcctctggaaccagcttctcagtggaatttcagatgctattcctggtcaattgcctttgctatgtgctatcctttaataaattctgtttctcctcatatccacctgagtcattctctgtaacctgcaaataagaactctgcctggtagatgaccctaggctctgccacttgtcagttgtccagagtcacacagctggtgagtgggtaagcccaactccctggactgccccacctgccccactgtctacccgaggagtcctggatgaagctggtgagtgccacgctgccaggtgtggcagccagaacagggatcttggagtgagtaggccaaagggtgagtaaactctaaatgggctgagagcaaaaagcatgtttttggggggaagagatgttctaccaagcctgactctttgggcaaggagagctaggaatggtttcagggccagggaccccagcctctggctctgagctgacagcaataaggatcccaaaaaatgagcacttagcagcaattaattgctaagatgcaaagaaaaattgttttgaatattaaaattatagctataacactattaggagcgtgattcagagtttatggaaacattatttatattgatttattcccagagccatcaagactccttgaaaataattaatgttgacatttccattgctgaagctaaatgttgatatcatataatgaaaattatatgcttgggatgggctgtgctctagaaagcattaaaacaaataccaacatctacagatccctccctacccccattactaatgacccagtaaccaatgggcagggctctgaggctcttcacctacaggcctctagcccagcatagccatcagcccatctgaggactctcagaagcaagggccagcaccccagggtaagcatggggctcatccagggccatgagccaggaggtgggccaggatctagacaggaagcccctttggccagatcctggtagtgactgagccactgaattgctgctggcctcaagaactgagggaaggagaaggacaagaggaggtgaggggagtgatttggctgtgactcactcaaaatctcatcttgaattgtaataatccccacatgtcaagggcgggaccaggtggagataattggatcatgggggcagtttcccccatgctgttcttgtgatagtgagttctcacaagatgtgatggttttataaggggcttcccccttccctcactctcattctctttcctgccgccatgtgaagaaggacgtgtttgcttccctttctgccatgtttgtaagtttcctgaggctttgccagccatgcaaaactgtgagtcaattaaacctcttttctttat

SEQ ID NO: 9584 - RNA, 1704 nt, Homo sapiens
  source 1..1704: mol_type = other RNA
agtttgggatggagagaggagaaaaaaagaagtgggtttccattcacttccattttctaactgatcattagttagagaacctttggaaaggtttagctcagttttttcttccaacttatcaggttcctcaagaaattcactgccttgagatgactttgataacccatccaaatccagtgacttaaaaccgttattacaagggctcttgctgttgtctgactctgacatcattgaatccaactcagagattttgtcaaggtaagcagcatccatcgatgcttcactggatgttcttgtccggttcatttcaaaagagcgaatagaattcaaccttttggataaacataagcctgatttctcactcaattttgaagatatttctccaacagaatttgctatcgtgttcccctctgaactttcaaaatctaagttttgggcatagcttgtggaacaacagtcccaaaatcctgtctttggggaagaaaaacattctgatttcttttcattttcacttctacttatatcatcttctgaagaatctttattagaaacatttgaagaatcacaaaaatcatcaaacaccaattttctgagatggtttgagtgctttttggaacctcctgcttggaccacagagctctctctattttctggagtactgagctgaaggcaactaagggacaaaggagtacaaggagctggaagatcataaagttcttcatctttgtagggtacacagtcacttggtttattcccccattctctttccaaataagtatccatacttgtatctgtcacatctaacattacttctacctgttcttgatataggtctttgttcttagaacagttaaggtctgctttgctggtactttcctgccttgcagaactggtgtcacacagtctgctgctggaaggcttcgctaggtgagaagaactggaggtggatgagccaggctgctttctggcactatcgccttgattctttgacaccacatcctcctcactgcctttgctccctttgccatctgcagaaagtgctgtctggcaaatggaattcatagcttctttctcttcacttgaattttttagctgtgcaacttgagattctagttcctctatatacttatcacttcgttccagggctttcttgaggcgattggtttcacgctcatactgttctactttggactgaagagcagcaactgcaaaccttccaaacttttgaggtgatctgttatcaacttcagccttcagtcgtaaattctccctcaccagaccaccattttccaatttcaattttttatttgcctcctttagcttatccacatcatctttcactttttcatagatttcattagctgttctgagttttttcttccactctgctacagtttctgggttaattttacttggattatctgtgactagatgtttgtcttcattttggttgccctgcaccaaggttaaaggatccagaatagttttgatctgtgactccaagctgagatttttactcttaagctcttctacttctttctgtaaacaatctatttcgtcctcatattctttgtgtagtaattcaagtctagttttccgaagatgcttcctgaccgtatggcttagcataggttcactttcacttgttcctcaatgaattcttcctgagagctcttcactgatgctctggttaccttctttgta

SEQ ID NO: 9585 - RNA, 1895 nt, Homo sapiens
  source 1..1895: mol_type = other RNA
agtttgggatggagagaggagaaaaaaagaagtgggtttccattcacttccattttctaactgatcattagttagagaacctttggaaaggtttagctcagttttttcttccaacttatcaggttcctcaagaaattcactgccttgagatgactttgataacccatccaaatccagtgacttaaaaccgttattacaagggctcttgctgttgtctgactctgacatcattgaatccaactcagagattttgtcaaggtaagcagcatccatcgatgcttcactggatgttcttgtccggttcatttcaaaagagcgaatagaattcaaccttttggataaacataagcctgatttctcactcaattttgaagatatttctccaacagaatttgctatcgtgttcccctctgaactttcaaaatctaagttttgggcatagcttgtggaacaacagtcccaaaatcctgtctttggggaagaaaaacattctgatttcttttcattttcacttctacttatatcatcttctgaagaatctttattagaaacatttgaagaatcacaaaaatcatcaaacaccaattttctgagatggtttgagtgctttttggaacctcctgcttggaccacagagctctctctattttctggagtactgagctgaaggcaactaagggacaaaggagtacaaggagctggaagatcataaagttcttcatctttgtagggtacacagtcacttggtttattcccccattctctttccaaataagtatccatacttgtatctgtcacatctaacattacttctacctgttcttgatataggtctttgttcttagaacagttaaggtctgctttgctggtactttcctgccttgcagaactggtgtcacacagtctgctgctggaaggcttcgctaggtgagaagaactggaggtggatgagccaggctgctttctggcactatcgccttgattctttgacaccacatcctcctcactgcctttgctccctttgccatctgcagaaagtgctgtctggcaaatggaattcatagcttctttctcttcacttgaattttttagctgtgcaacttgagattctagttcctctatatacttatcacttcgttccagggctttcttgaggcgattggtttcacgctcatactgttctactttggactgaagagcagcaactgcaaaccttccaaacttttgaggtgatctgttatcaacttcagccttcagtcgtaaattctccctcaccagaccaccattttccaatttcaattttttatttgcctcctttagcttatccacatcatctttcactttttcatagatttcattagctgttctgagttttttcttccactctgctacagtttctgggttaattttacttggattatctgtgactagatgtttgtcttcattttggttgccctgcaccaaggttaaaggatccagaatagttttgatctgtgactccaagctgagatttttactcttaagctcttctacttctttctgtaaacaatctatttcgtcctcatattctttgtgtagtaattcaagtctagttttccgaagatgcttcctgaccgtatggcttagcataggttcactttcacttgttcctcctataatttctttgcaaggattttcaggagtgatggggactctgcaagctggacactggctattattcttcaaccacaaatcaatacaaatcgaacaaaatacatggttgttgatgcatatgacaggctgacgtaccttccccaagcaaatgtggcacgtgatgggcagagtgagcgacaatgtaacattctgcacggtctgagccatggcagcgttcagaatcccgccaacacggaagtccc

SEQ ID NO: 9586 - RNA, 1769 nt, Homo sapiens
  source 1..1769: mol_type = other RNA
agtttgggatggagagaggagaaaaaaagaagtgggtttccattcacttccattttctaactgatcattagttagagaacctttggaaaggtttagctcagttttttcttccaacttatcaggttcctcaagaaattcactgccttgagatgactttgataacccatccaaatccagtgacttaaaaccgttattacaagggctcttgctgttgtctgactctgacatcattgaatccaactcagagattttgtcaaggtaagcagcatccatcgatgcttcactggatgttcttgtccggttcatttcaaaagagcgaatagaattcaaccttttggataaacataagcctgatttctcactcaattttgaagatatttctccaacagaatttgctatcgtgttcccctctgaactttcaaaatctaagttttgggcatagcttgtggaacaacagtcccaaaatcctgtctttggggaagaaaaacattctgatttcttttcattttcacttctacttatatcatcttctgaagaatctttattagaaacatttgaagaatcacaaaaatcatcaaacaccaattttctgagatggtttgagtgctttttggaacctcctgcttggaccacagagctctctctattttctggagtactgagctgaaggcaactaagggacaaaggagtacaaggagctggaagatcataaagttcttcatctttgtagggtacacagtcacttggtttattcccccattctctttccaaataagtatccatacttgtatctgtcacatctaacattacttctacctgttcttgatataggtctttgttcttagaacagttaaggtctgctttgctggtactttcctgccttgcagaactggtgtcacacagtctgctgctggaaggcttcgctaggtgagaagaactggaggtggatgagccaggctgctttctggcactatcgccttgattctttgacaccacatcctcctcactgcctttgctccctttgccatctgcagaaagtgctgtctggcaaatggaattcatagcttctttctcttcacttgaattttttagctgtgcaacttgagattctagttcctctatatacttatcacttcgttccagggctttcttgaggcgattggtttcacgctcatactgttctactttggactgaagagcagcaactgcaaaccttccaaacttttgaggtgatctgttatcaacttcagccttcagtcgtaaattctccctcaccagaccaccattttccaatttcaattttttatttgcctcctttagcttatccacatcatctttcactttttcatagatttcattagctgttctgagttttttcttccactctgctacagtttctgggttaattttacttggattatctgtgactagatgtttgtcttcattttggttgccctgcaccaaggttaaaggatccagaatagttttgatctgtgactccaagctgagatttttactcttaagctcttctacttctttctgtaaacaatctatttcgtcctcatattctttgtgtagtaattcaagtctagttttccgaagatgcttcctgaccgtatggcttagcataggttcactttcacttgttcctccttccccaagcaaatgtggcacgtgatgggcagagtgagcgacaatgtaacattctgcacggtctgagccatggcagcgttcagaatcccgccaacacggaagtcccgccgacctac

SEQ ID NO: 9587 - RNA, 3806 nt, Homo sapiens
  source 1..3806: mol_type = other RNA
agtttgggatggagagaggagagatccattatctctaatttccttggaagggattcagggaacgggatggggttgctaggagacggagacgtgagggaagaaggaacgatgtaagaagtcatccaggtggggctggaaagggggtggacaggagcatttcaggtgaatggagaaagggaatggtgggggtggtccacacaggggccctgaagggagaggagggcagctgagaagggagctattgggttggaggacgagggggttgtaggcatgtgcttgtgcaggccattgctgagagccttggtgagcgtgcaggtccttaacaaatgctttacgatgctgtgtatgtgtctgtctagcctgtgaagctggttagagtggatgaatgtgtttttgtgactgttgaggcagagtgtgcatacaggtatgaggggatggcaacagagaaagaaacagaaacagaaacaggaggaatataaaatcgcctttagaggtatgaggcttagggcattttttactaagtagatactcaaaggtgtacgctcttgacaggaataaagcctgtcctttggcataaggtacagtgatggctgctatgaagggtgaagttctcggcagtgggaaacttgtcccacttttccatggcatgcacccaccctgggactaaaccctgagcagaagtgacagggacccatgagtttgctccctccccaactgccgcattatccaagccagactcccacttgagacaacccactcatggccagcacaccaggaggcacgacaggacagtaactgcccagcatcccctgccatgaggcagggatgcgtcccctctttccctcctccctccaccagggtctaagagctggaggtctgggccctgtgttccagtcacacctcatgataagaacacattttgtgacaacagtcatacatatcatataaatatatttgttcaaactacaaagggatggatatcagggggaagcttttattgctgtggggggacctggagagggaggggggccttggaaatggggatacctgggaccacttgttccccccattcctcacagaaggcacaaatacattatttctttccatgtgaggagatgcgaggagaggatacagaatacaggaatcctcaaaaatacaaaaaacccctccaaactgaatacctaaggttatggaaaaggctagggtggggcacagaagtcaatgggggaacagaaagaggaaccaatgaaactgagaaccaaaagggacctgagaggccatgatgtccatgctgctgcctctgtgcagaccccagagaaaactcaggtaaaccaacggaaactccaaataagagagggtagggtgccccaggaattggctttggggcatcagacaagggagtgtgagtgtgagtgtgtgtgtgcagtggctgtgtatcagaagcaaccagggctaggagtggacgattctattcccacaggggaaggcctcctccatcccggttcctccaaaaccactttcaggggataaattcagccactgcttccgaacaggacccctccctgggacaaaagagccaggtaggagaggatgaagtgagaaatcttgggatgaaaacagggcacacagaagcagttcttagggaacagaatatcatggagcccagtgtgatagaaaatgggcatgaaacctaagtgtatgcatgtgtgtgagtgtgtgtgtgcatgagtgtgtatttgtgcatgtacgagggagtaagatcactcaaaggtgaaggggtcctgggtgctgaaaaagaagtgtccatccatgtggtcctccagggcatccttgtcactctcagcaggaaagcgctccttacagataggacactccttccatgtgggggtggcagggcccccagtgctggtttctgacagggtacccactgtaaagccactggccatgtcatagaaggcactgcccagttcaggaagcagtaagttggcctcctcacccccactctgcacagctgccatcaggactgacttctcatcttcagcctccgagtcagagctactgtcctcagctggcccagagaggtgaggagaaatgggagccggctggctgatgacaacaaggggagaagcctctcgaggcccagcaggagaggagcctgggtctccacgctcacaaaggccatagggtgggagcctcatgtcttctggggactcgtcctctgagtctgtcagagctgccgggcagctcagccccacagcggcctcctcatcctctgtggtggcatcctcattccacttctcatctgccaccttctccaggcgggcctctagctttctcatgtactctagcaattcctgtttctcctcctgtaactgctccttttccttctggagcacacgcagggctgaccgcagctctgtcagctcccgcttactttctgacaactgtaccaggctagaatccttctcccgggccagctcagtcttgaacacttggttttgggtcctctcctcctgaactgccttctccaatcgaagtatctctgcactcagcttcaggatcttgtccttctctgcctccacactctgcagcagccctgcccgctccttgctccattggcatttttcttccttcaagtgcaaaccgagctcagccagcctgccgttaacttcagccacttccaggcggctgcggtgtagttcggctatggtgcggtccctggctgctgctgcactggccaactcctccccaagaagggtggctttctgctggcttgaggctgcaagctcctgggcccctcgaagctgctccttcaagggctccagctcggccacccgctgctgggcctggcctagggtgtccttcatctgggccaccttgtctttcagtcgctgagcctgagcactctgctcctcttgccagctcttcgcctccttcaggtccaaatttaagtgatggttctcctgttgtgccacttggagctcagcctcactttgctccttgtctgcttgtacttctttcagttgcccaaggagcttctcttgttcccgagtcagggccttcactgtgtctctaagcctgtccagctccacttccttcgtcagcactttctcactgatggtctggatgtcatcctctagctccaggatgcgtgccacatggtctccctgttgccggctcaggatgtccctctcttctgtgatctccccatgggaccgggaaatccccttgtactgttccatcagctccgtgtgctcctgcctggcagttgccagagccctctcgagctcctgcactcggctcctcagctctgtcacctgtccctccagctgtagcttcagctgcatcaggtcattccgttcttgctggctctcatcgagctggttctgtaacacagttgccttggggacaaccagcaggatgtcagagcccccatcagcctcctccagggtcaccagttcatccatgggccttggctctcggaactggaaaggggggctctgcccacacacctggccctggcggttcacatatcggaactggtagagctgagctcctggtttgggcaggtagctggcttgaagatgccaatccagtcactggcactgggcatggtgcctgggggaagggtgtagtgacattccaccttggtgttggggatgtaggtccgggctacattgagaaagttgactccaccacgggatggtgcccggcttagtggtgattcttccatcctggccttgagatatctgtcctcccaacagacggatcagctgttcccctcacctttcaccaacaacaaaaac

SEQ ID NO: 9588 - RNA, 3909 nt, Homo sapiens
  source 1..3909: mol_type = other RNA
agtttgggatggagagaggagagatccattatctctaatttccttggaagggattcagggaacgggatggggttgctaggagacggagacgtgagggaagaaggaacgatgtaagaagtcatccaggtggggctggaaagggggtggacaggagcatttcaggtgaatggagaaagggaatggtgggggtggtccacacaggggccctgaagggagaggagggcagctgagaagggagctattgggttggaggacgagggggttgtaggcatgtgcttgtgcaggccattgctgagagccttggtgagcgtgcaggtccttaacaaatgctttacgatgctgtgtatgtgtctgtctagcctgtgaagctggttagagtggatgaatgtgtttttgtgactgttgaggcagagtgtgcatacaggtatgaggggatggcaacagagaaagaaacagaaacagaaacaggaggaatataaaatcgcctttagaggtatgaggcttagggcattttttactaagtagatactcaaaggtgtacgctcttgacaggaataaagcctgtcctttggcataaggtacagtgatggctgctatgaagggtgaagttctcggcagtgggaaacttgtcccacttttccatggcatgcacccaccctgggactaaaccctgagcagaagtgacagggacccatgagtttgctccctccccaactgccgcattatccaagccagactcccacttgagacaacccactcatggccagcacaccaggaggcacgacaggacagtaactgcccagcatcccctgccatgaggcagggatgcgtcccctctttccctcctccctccaccagggtctaagagctggaggtctgggccctgtgttccagtcacacctcatgataagaacacattttgtgacaacagtcatacatatcatataaatatatttgttcaaactacaaagggatggatatcagggggaagcttttattgctgtggggggacctggagagggaggggggccttggaaatggggatacctgggaccacttgttccccccattcctcacagaaggcacaaatacattatttctttccatgtgaggagatgcgaggagaggatacagaatacaggaatcctcaaaaatacaaaaaacccctccaaactgaatacctaaggttatggaaaaggctagggtggggcacagaagtcaatgggggaacagaaagaggaaccaatgaaactgagaaccaaaagggacctgagaggccatgatgtccatgctgctgcctctgtgcagaccccagagaaaactcaggtaaaccaacggaaactccaaataagagagggtagggtgccccaggaattggctttggggcatcagacaagggagtgtgagtgtgagtgtgtgtgtgcagtggctgtgtatcagaagcaaccagggctaggagtggacgattctattcccacaggggaaggcctcctccatcccggttcctccaaaaccactttcaggggataaattcagccactgcttccgaacaggacccctccctgggacaaaagagccaggtaggagaggatgaagtgagaaatcttgggatgaaaacagggcacacagaagcagttcttagggaacagaatatcatggagcccagtgtgatagaaaatgggcatgaaacctaagtgtatgcatgtgtgtgagtgtgtgtgtgcatgagtgtgtatttgtgcatgtacgagggagtaagatcactcaaaggtgaaggggtcctgggtgctgaaaaagaagtgtccatccatgtggtcctccagggcatccttgtcactctcagcaggaaagcgctccttacagataggacactccttccatgtgggggtggcagggcccccagtgctggtttctgacagggtacccactgtaaagccactggccatgtcatagaaggcactgcccagttcaggaagcagtaagttggcctcctcacccccactctgcacagctgccatcaggactgacttctcatcttcagcctccgagtcagagctactgtcctcagctggcccagagaggtgaggagaaatgggagccggctggctgatgacaacaaggggagaagcctctcgaggcccagcaggagaggagcctgggtctccacgctcacaaaggccatagggtgggagcctcatgtcttctggggactcgtcctctgagtctgtcagagctgccgggcagctcagccccacagcggcctcctcatcctctgtggtggcatcctcattccacttctcatctgccaccttctccaggcgggcctctagctttctcatgtactctagcaattcctgtttctcctcctgtaactgctccttttccttctggagcacacgcagggctgaccgcagctctgtcagctcccgcttactttctgacaactgtaccaggctagaatccttctcccgggccagctcagtcttgaacacttggttttgggtcctctcctcctgaactgccttctccaatcgaagtatctctgcactcagcttcaggatcttgtccttctctgcctccacactctgcagcagccctgcccgctccttgctccattggcatttttcttccttcaagtgcaaaccgagctcagccagcctgccgttaacttcagccacttccaggcggctgcggtgtagttcggctatggtgcggtccctggctgctgctgcactggccaactcctccccaagaagggtggctttctgctggcttgaggctgcaagctcctgggcccctcgaagctgctccttcaagggctccagctcggccacccgctgctgggcctggcctagggtgtccttcatctgggccaccttgtctttcagtcgctgagcctgagcactctgctcctcttgccagctcttcgcctccttcaggtccaaatttaagtgatggttctcctgttgtgccacttggagctcagcctcactttgctccttgtctgcttgtacttctttcagttgcccaaggagcttctcttgttcccgagtcagggccttcactgtgtctctaagcctgtccagctccacttccttcgtcagcactttctcactgatggtctggatgtcatcctctagctccaggatgcgtgccacatggtctccctgttgccggctcaggatgtccctctcttctgtgatctccccatgggaccgggaaatccccttgtactgttccatcagctccgtgtgctcctgcctggcagttgccagagccctctcgagctcctgcactcggctcctcagctctgtcacctgtccctccagctgtagcttcagctgcatcaggtcattccgttcttgctggctctcatcgagctggttctgtaacacagttgccttggggacaaccagcaggatgtcagagcccccatcagcctcctccagggtcaccagttcatccatgggccttggctctcggaactggaaaggggggctctgcccacacacctggccctggcggttcacatatcggaactggtagagctgagctcctggtttgggcaggtagctggcttggaactggacactggtgtgaatgggggaaccatcagttgtactttcaggcacggaagaccacacaaatgtgtggtaatcccgaacacaggcagcctccaccttgaagatgccaatccagtcactggcactgggcatggtgcctgggggaagggtgtagtgacattccaccttggtgttggggatgtaggtccgggctacattgagaaagttgactccaccacgggatggtgcccggcttagtggtgattcttccatcctggccttgagatatctgtcctcccaacagacggatcagctgttcccctcacctttcaccaacaacaaaaac

SEQ ID NO: 9589 - RNA, 3654 nt, Homo sapiens
  source 1..3654: mol_type = other RNA
agtttgggatggagagaggagagatccattatctctaatttccttggaagggattcagggaacgggatggggttgctaggagacggagacgtgagggaagaaggaacgatgtaagaagtcatccaggtggggctggaaagggggtggacaggagcatttcaggtgaatggagaaagggaatggtgggggtggtccacacaggggccctgaagggagaggagggcagctgagaagggagctattgggttggaggacgagggggttgtaggcatgtgcttgtgcaggccattgctgagagccttggtgagcgtgcaggtccttaacaaatgctttacgatgctgtgtatgtgtctgtctagcctgtgaagctggttagagtggatgaatgtgtttttgtgactgttgaggcagagtgtgcatacaggtatgaggggatggcaacagagaaagaaacagaaacagaaacaggaggaatataaaatcgcctttagaggtatgaggcttagggcattttttactaagtagatactcaaaggtgtacgctcttgacaggaataaagcctgtcctttggcataaggtacagtgatggctgctatgaagggtgaagttctcggcagtgggaaacttgtcccacttttccatggcatgcacccaccctgggactaaaccctgagcagaagtgacagggacccatgagtttgctccctccccaactgccgcattatccaagccagactcccacttgagacaacccactcatggccagcacaccaggaggcacgacaggacagtaactgcccagcatcccctgccatgaggcagggatgcgtcccctctttccctcctccctccaccagggtctaagagctggaggtctgggccctgtgttccagtcacacctcatgataagaacacattttgtgacaacagtcatacatatcatataaatatatttgttcaaactacaaagggatggatatcagggggaagcttttattgctgtggggggacctggagagggaggggggccttggaaatggggatacctgggaccacttgttccccccattcctcacagaaggcacaaatacattatttctttccatgtgaggagatgcgaggagaggatacagaatacaggaatcctcaaaaatacaaaaaacccctccaaactgaatacctaaggttatggaaaaggctagggtggggcacagaagtcaatgggggaacagaaagaggaaccaatgaaactgagaaccaaaagggacctgagaggccatgatgtccatgctgctgcctctgtgcagaccccagagaaaactcaggtaaaccaacggaaactccaaataagagagggtagggtgccccaggaattggctttggggcatcagacaagggagtgtgagtgtgagtgtgtgtgtgcagtggctgtgtatcagaagcaaccagggctaggagtggacgattctattcccacaggggaaggcctcctccatcccggttcctccaaaaccactttcaggggataaattcagccactgcttccgaacaggacccctccctgggacaaaagagccaggtaggagaggatgaagtgagaaatcttgggatgaaaacagggcacacagaagcagttcttagggaacagaatatcatggagcccagtgtgatagaaaatgggcatgaaacctaagtgtatgcatgtgtgtgagtgtgtgtgtgcatgagtgtgtatttgtgcatgtacgagggagtaagatcactcaaaggtgaaggggtcctgggtgctgaaaaagaagtgtccatccatgtggtcctccagggcatccttgtcactctcagcaggaaagcgctccttacagataggacactccttccatgtgggggtggcagggcccccagtgctggtttctgacagggtacccactgtaaagccactggccatgtcatagaaggcactgcccagttcaggaagcagtaagttggcctcctcacccccactctgcacagctgccatcaggactgacttctcatcttcagcctccgagtcagagctactgtcctcagctggcccagagaggtgaggagaaatgggagccggctggctgatgacaacaaggggagaagcctctcgaggcccagcaggagaggagcctgggtctccacgctcacaaaggccatagggtgggagcctcatgtcttctggggactcgtcctctgagtctgtcagagctgccgggcagctcagccccacagcggcctcctcatcctctgtggtggcatcctcattccacttctcatctgccaccttctccaggcgggcctctagctttctcatgtactctagcaattcctgtttctcctcctgtaactgctccttttccttctggagcacacgcagggctgaccgcagctctgtcagctcccgcttactttctgacaactgtaccaggctagaatccttctcccgggccagctcagtcttgaacacttggttttgggtcctctcctcctgaactgccttctccaatcgaagtatctctgcactcagcttcaggatcttgtccttctctgcctccacactctgcagcagccctgcccgctccttgctccattggcatttttcttccttcaagtgcaaaccgagctcagccagcctgccgttaacttcagccacttccaggcggctgcggtgtagttcggctatggtgcggtccctggctgctgctgcactggccaactcctccccaagaagggtggctttctgctggcttgaggctgcaagctcctgggcccctcgaagctgctccttcaagggctccagctcggcctcactttgctccttgtctgcttgtacttctttcagttgcccaaggagcttctcttgttcccgagtcagggccttcactgtgtctctaagcctgtccagctccacttccttcgtcagcactttctcactgatggtctggatgtcatcctctagctccaggatgcgtgccacatggtctccctgttgccggctcaggatgtccctctcttctgtgatctccccatgggaccgggaaatccccttgtactgttccatcagctccgtgtgctcctgcctggcagttgccagagccctctcgagctcctgcactcggctcctcagctctgtcacctgtccctccagctgtagcttcagctgcatcaggtcattccgttcttgctggctctcatcgagctggttctgtaacacagttgccttggggacaaccagcaggatgtcagagcccccatcagcctcctccagggtcaccagttcatccatgggccttggctcttggaactggacactggtgtgaatgggggaaccatcagttgtactttcaggcacggaagaccacacaaatgtgtggtaatcccgaacacaggcagcctccaccttgaagatgccaatccagtcactggcactgggcatggtgcctgggggaagggtgtagtgacattccaccttggtgttggggatgtaggtccgggctacattgagaaagttgactccaccacgggatggtgcccggcttagtggtgattcttccatcctggccttgagatatctgtcctcccaacagacggatcagctgttcccctcacctttcaccaacaacaaaaac

SEQ ID NO: 9590 - RNA, 58 nt, Homo sapiens
  source 1..58: mol_type = other RNA
ataatacaacctgctaagtgctaggacacttagcaggttgtattatatccatccgagt

SEQ ID NO: 9591 - RNA, 70 nt, Homo sapiens
  source 1..70: mol_type = other RNA
atacatgtcagattgtatgccagtctggagggattttgtaggcatacaatctgacatgtatttaagtgat

SEQ ID NO: 9592 - RNA, 21 nt, Homo sapiens
  source 1..21: mol_type = other RNA
atacccatagcttagctccca

SEQ ID NO: 9593 - RNA, 4474 nt, Homo sapiens
  source 1..4474: mol_type = other RNA
atacccatagcttagctcccacatatcaatgagaacataggttgtttggttttccattcctgagttacttaacttagaataatagtttccaacaataaaaacaaagataaatagatgggacttaattaaactaaagagcttttgcatggtaaaagcaacagtcagcagagtaaacagacaacgcacagagtgggagaaaatcttcacaatctatacatcagacaaaggactaatatccagaatctacaacaaactcaaacaaatcagtaagaaaaaaacaaacaatcccatcaaaaagtgggttaaggacatgaatagacaattctcaaaagaagatatacaaatggccaacaaagtatgaaaaaatgctcaacatcactaatgatcagggaaatgcaaataaaaactacagtgcgatacccccttactcctgcaagaacggccataaccaaaaaaatcaaaaaacagtagatgttggcatgcatgcggcaatcatggaacacttccacactgctggtgggaatgtaaactattagagccaccatggaaaacagtgtggaaattccttagaactaaaagtagaactaccatttgatccagcaatcccattactgggtatctacccagaggaaaagaagtcattattcaaaaaaagatacttgcacgcacatgtttatagcagcacaattcacaactgcaaaatcgtggaaccaacccaaatgcccatcagtcaacaagtggtatatatatatatacaatggaatactactcagccataaaaaggaatcaattagcagtatttgcaatgatctggttgatcaatatcttaagaaaggtggttaagctttggttacagcaatggccgatagagaagattatggctgtatcagacacaagtgagggtcccttcccttttccttgcttttattcttgttatttttttctacctaacattattttagctacttacttgtttcttacctgtcactccacctgggccaggactgttttttctacccatccgtcctcagcacccactgctgtgcttgatatacagtaagtgcttggcaaatgttgttgaatgcacaaatgcatgcaccgctggccttggagactaaggaggagatgggtacaactattgttctctgcctcattggattttagctttggtcatgatagcagttggctgtggtcttcctacagataacagcagacagggtctggacggaaggagagaaatgggcttttgggttccaagttctgtcagtgttgggtgactgaagtcgtgcacagaggcctctctgagggagaagccatggccatgccaccccctggcttccctgcagcttgaggcaggaggtaaccagccattatggggcaggatccctataggccaaaatgtggagactttatttttttcctgggatgccaacacctagttctctggttttccccacttagttaatttttgtgttaggaaaggccacctcctcagcctaccttctcttccccggcaatgggcacatggctcatttctgggctctctgtgctctccctggagagtgggggtgcagaggacactgctttctgctgcaggcgccatgtttagttggtctcactttgagatgctcatttccctctgccttctgtcagcccagatgtgaggacccagggtctccgcagggtgtgcactgtcatggcctctctgctctgccacatcaggcccatctccacccgtgctgtggtccatctgcagtggtgactctctctcactctctttatggggccactcccccacctaaattcctttgaggtgatttcaactggggtcagaatagagaggggagaaggaaaggtgtatgttcagctcatcagatttaactggaagctctcaaggctactttaaaaatcataaaagccattcccaataagcttgtttgttttaaaggaaatctcctttccaaatcactgtagatagtaaacagaagaagttgaaaaaaccaaataaaaacaggaaatatgatgaaagaatgtttcgatgtaacaattagtaaaagaatttgagctaccttgttaaatggcaaagtctatttattatgttgttaaagacaactgaaacaaatggcatttaaaaactccagatgagatgataaggcaaagcaatgccagatgaattcatcaagataaaaagcagtatggcaatgtttttatcaaagtagaattcaagtcatgaagcattcaacaggaagattattttatattgataacaggtacaggctatgaggggaaagctttgcaaagcaacaacagcaaaacagaaagcaaaaactattagaaggaagattagctatggaagaaaaagaaggctgtagagaattttaacaattattatgtttcaatcaacaaagaacaaacaggataaatcttaaaaagtggtcttgttattgttacagaaagtgatcattctttacactacaagggaaaactcaaaatctacaaaagagaaatttcacagacaacaatctctactatatccatacgtggggaacagaacaaaaaaactaggtctagactagaagacagagagaaaccatgtcagaccagagcacattgatggctcacggtgagtgacccatggcctaaaggtgcctgtttagggcccaggagccactcacacaggcagagcagcttactccgtatgaaccaccaccagcacccctccctgcccggtgatgtcacccggtgggctgggctggaacaagtccagatgcctttgcctcaccttggaagggccacgaggagcttcctcctctatccccaagttctccacttacacacagcacctgacacgaaggttggcaagtttcccccgggccatgactgcacaatggctacccccagcctctgtggcctccgagagagggctcctagacagattccagccctatagggggagggaagcaacactgcagttgaccttgaagagatcactgtagggggctatagaagggattgtgacatttattgttctgaaaatgccatcaaagacagttgtaaagtctagtctcatacacacttggcaagacatagccaaaagaggtaaatttgaaattagaaaaaatatcagcagttattacccagagcttgaaattctgacctgttacacagtaggatattcaacctccatttcagcgtatttaggtacttattaggtagattgcaaaattactagaaaaaaaattcctagaggacatcttgaaaatgataaagtagcaggaaaattacaaagatataacttatttacaaagtccatagagaagcgccattggaaagcttcaagttgaagataatttcatgaaaaacgcacttaaaacaaaaatggaattataatttttctgaactttggatactcttcaaatttccggaggtaccactcatgatgctcttttgctctaccagataaaaaacaaaacgtgaagaaagcaaaagccgcgccttggacagaccagctggccagggcatagccacaccactccatgatttctccaaaatagttggctgcagttacgtattcaaataagcctccccttggtattttgtatccagtatctcctggttttctgagattccttaggatatgatctgaatggatgtttatcaacatgcccgttaaccacaagccaaaaccacttgcggaagctcagcttggtgaggtggtggaaatcaccgctctgccattcactgcgtctagatgtcttgggccagctgtgtaactcttctgacctttcacatcttagggacatcctttctgcctcagagaacatggggaggcataaatcgtgtgatctgcacaggaactcaaaagcctgttcttcctctattagaaaacggggatctgttacccagtcatcagcatacactgcacaatggctcaagtatctgctttgcaaatagccgttacaggtacagaacataatcgccattgtacacgccaacagtggcataggctttcctcctcgcatcagaaatgggtaaattaagcaccgatgcccgtagtggacgaggaacatggccaggaggatgcagttgggcgcgctgcggagacgcggggcggactcgctggcgtactggtagagcggcagggccagcgagggcagctcctgcaccacccaggcggcccgcgccggcactcggagcctgtggctgggcagcgcgtggcggccgtacactgagttcgtctgacgattgcgcgcgaagaccgcgcagcccacggcgcactgcaggtaggcgagcgcggccagcaggcgctcctccgccacccccgtcgccgttgccatcgccagggctgggcagcgtgctccatgccccagaggccgcggcgggcaacatatagggcggcggcgcgggggcaggaggggcggctaccggaggggcggctaccggagtcccgcactgccgggactctgcagaaagg

SEQ ID NO: 9594 - RNA, 4117 nt, Homo sapiens
  source 1..4117: mol_type = other RNA
atacccatagcttagctcccacatatcaatgagaacataggttgtttggttttccattcctgagttacttaacttagaataatagtttccaacaataaaaacaaagataaatagatgggacttaattaaactaaagagcttttgcatggtaaaagcaacagtcagcagagtaaacagacaacgcacagagtgggagaaaatcttcacaatctatacatcagacaaaggactaatatccagaatctacaacaaactcaaacaaatcagtaagaaaaaaacaaacaatcccatcaaaaagtgggttaaggacatgaatagacaattctcaaaagaagatatacaaatggccaacaaagtatgaaaaaatgctcaacatcactaatgatcagggaaatgcaaataaaaactacagtgcgatacccccttactcctgcaagaacggccataaccaaaaaaatcaaaaaacagtagatgttggcatgcatgcggcaatcatggaacacttccacactgctggtgggaatgtaaactattagagccaccatggaaaacagtgtggaaattccttagaactaaaagtagaactaccatttgatccagcaatcccattactgggtatctacccagaggaaaagaagtcattattcaaaaaaagatacttgcacgcacatgtttatagcagcacaattcacaactgcaaaatcgtggaaccaacccaaatgcccatcagtcaacaagtggtatatatatatatacaatggaatactactcagccataaaaaggaatcaattagcagtatttgcaatgatctggttgatcaatatcttaagaaaggtggttaagctttggttacagcaatggccgatagagaagattatggctgtatcagacacaagtgagggtcccttcccttttccttgcttttattcttgttatttttttctacctaacattattttagctacttacttgtttcttacctgtcactccacctgggccaggactgttttttctacccatccgtcctcagcacccactgctgtgcttgatatacagtaagtgcttggcaaatgttgttgaatgcacaaatgcatgcaccgctggccttggagactaaggaggagatgggtacaactattgttctctgcctcattggattttagctttggtcatgatagcagttggctgtggtcttcctacagataacagcagacagggtctggacggaaggagagaaatgggcttttgggttccaagttctgtcagtgttgggtgactgaagtcgtgcacagaggcctctctgagggagaagccatggccatgccaccccctggcttccctgcagcttgaggcaggaggtaaccagccattatggggcaggatccctataggccaaaatgtggagactttatttttttcctgggatgccaacacctagttctctggttttccccacttagttaatttttgtgttaggaaaggccacctcctcagcctaccttctcttccccggcaatgggcacatggctcatttctgggctctctgtgctctccctggagagtgggggtgcagaggacactgctttctgctgcaggcgccatgtttagttggtctcactttgagatgctcatttccctctgccttctgtcagcccagatgtgaggacccagggtctccgcagggtgtgcactgtcatggcctctctgctctgccacatcaggcccatctccacccgtgctgtggtccatctgcagtggtgactctctctcactctctttatggggccactcccccacctaaattcctttgaggtgatttcaactggggtcagaatagagaggggagaaggaaaggtgtatgttcagctcatcagatttaactggaagctctcaaggctactttaaaaatcataaaagccattcccaataagcttgtttgttttaaaggaaatctcctttccaaatcactgtagatagtaaacagaagaagttgaaaaaaccaaataaaaacaggaaatatgatgaaagaatgtttcgatgtaacaattagtaaaagaatttgagctaccttgttaaatggcaaagtctatttattatgttgttaaagacaactgaaacaaatggcatttaaaaactccagatgagatgataaggcaaagcaatgccagatgaattcatcaagataaaaagcagtatggcaatgtttttatcaaagtagaattcaagtcatgaagcattcaacaggaagattattttatattgataacaggtacaggctatgaggggaaagctttgcaaagcaacaacagcaaaacagaaagcaaaaactattagaaggaagattagctatggaagaaaaagaaggctgtagagaattttaacaattattatgtttcaatcaacaaagaacaaacaggataaatcttaaaaagtggtcttgttattgttacagaaagtgatcattctttacactacaagggaaaactcaaaatctacaaaagagaaatttcacagacaacaatctctactatatccatacgtggggaacagaacaaaaaaactaggtctagactagaagacagagagaaaccatgtcagaccagagcacattgatggctcacggtgagtgacccatggcctaaaggtgcctgtttagggcccaggagccactcacacaggcagagcagcttactccgtatgaaccaccaccagcacccctccctgcccggtgatgtcacccggtgggctgggctggaacaagtccagatgcctttgcctcaccttggaagggccacgaggagcttcctcctctatccccaagttctccacttacacacagcacctgacacgaaggttggcaagtttcccccgggccatgactgcacaatggctacccccagcctctgtggcctccgagagagggctcctagacagattccagccctatagggggagggaagcaacactgcagttgaccttgaagagatcactgtagggggctatagaagggattgtgacatttattgttctgaaaatgccatcaaagacagttgtaaagtctagtctcatacacacttggcaagacatagccaaaagaggtaaatttgaaattagaaaaaatatcagcagttattacccagagcttgaaattctgacctgttacacagtaggatattcaacctccatttcagcgtatttaggtacttattaggtagattgcaaaattactagaaaaaaaattcctagaggacatcttgaaaatgataaagtagcaggaaaattacaaagatataacttatttacaaagtccatagagaagcgccattggaaagcttcaagttgaagataatttcatgaaaaacgcacttaaaacaaaaatggaattataatttttctgaactttggatactcttcaaatttccggaggtaccactcatgatgctcttttgctctaccagataaaaaacaaaacgtgaagaaagcaaaagccgcgccttggacagaccagctggccagggcatagccacaccactccatgatttctccaaaatagttggctgcagttacgtattcaaataagcctccccttggtattttgtatccagtatctcctggttttctgagattccttaggatatgatctgaatggatgtttatcaacatgcccgttaaccacaagccaaaaccgatgcccgtagtggacgaggaacatggccaggaggatgcagttgggcgcgctgcggagacgcggggcggactcgctggcgtactggtagagcggcagggccagcgagggcagctcctgcaccacccaggcggcccgcgccggcactcggagcctgtggctgggcagcgcgtggcggccgtacactgagttcgtctgacgattgcgcgcgaagaccgcgcagcccacggcgcactgcaggtaggcgagcgcggccagcaggcgctcctccgccacccccgtcgccgttgccatcgccagggctgggcagcgtgctccatgccccagaggccgcggcgggcaacatatagggcggcggcgcgggggcaggaggggcggctaccggaggggcggctaccggagtcccgcactgccgggactctgcagaaagg

SEQ ID NO: 9595 - RNA, 4284 nt, Homo sapiens
  source 1..4284: mol_type = other RNA
atacccatagcttagctcccacatatcaatgagaacataggttgtttggttttccattcctgagttacttaacttagaataatagtttccaacaataaaaacaaagataaatagatgggacttaattaaactaaagagcttttgcatggtaaaagcaacagtcagcagagtaaacagacaacgcacagagtgggagaaaatcttcacaatctatacatcagacaaaggactaatatccagaatctacaacaaactcaaacaaatcagtaagaaaaaaacaaacaatcccatcaaaaagtgggttaaggacatgaatagacaattctcaaaagaagatatacaaatggccaacaaagtatgaaaaaatgctcaacatcactaatgatcagggaaatgcaaataaaaactacagtgcgatacccccttactcctgcaagaacggccataaccaaaaaaatcaaaaaacagtagatgttggcatgcatgcggcaatcatggaacacttccacactgctggtgggaatgtaaactattagagccaccatggaaaacagtgtggaaattccttagaactaaaagtagaactaccatttgatccagcaatcccattactgggtatctacccagaggaaaagaagtcattattcaaaaaaagatacttgcacgcacatgtttatagcagcacaattcacaactgcaaaatcgtggaaccaacccaaatgcccatcagtcaacaagtggtatatatatatatacaatggaatactactcagccataaaaaggaatcaattagcagtatttgcaatgatctggttgatcaatatcttaagaaaggtggttaagctttggttacagcaatggccgatagagaagattatggctgtatcagacacaagtgagggtcccttcccttttccttgcttttattcttgttatttttttctacctaacattattttagctacttacttgtttcttacctgtcactccacctgggccaggactgttttttctacccatccgtcctcagcacccactgctgtgcttgatatacagtaagtgcttggcaaatgttgttgaatgcacaaatgcatgcaccgctggccttggagactaaggaggagatgggtacaactattgttctctgcctcattggattttagctttggtcatgatagcagttggctgtggtcttcctacagataacagcagacagggtctggacggaaggagagaaatgggcttttgggttccaagttctgtcagtgttgggtgactgaagtcgtgcacagaggcctctctgagggagaagccatggccatgccaccccctggcttccctgcagcttgaggcaggaggtaaccagccattatggggcaggatccctataggccaaaatgtggagactttatttttttcctgggatgccaacacctagttctctggttttccccacttagttaatttttgtgttaggaaaggccacctcctcagcctaccttctcttccccggcaatgggcacatggctcatttctgggctctctgtgctctccctggagagtgggggtgcagaggacactgctttctgctgcaggcgccatgtttagttggtctcactttgagatgctcatttccctctgccttctgtcagcccagatgtgaggacccagggtctccgcagggtgtgcactgtcatggcctctctgctctgccacatcaggcccatctccacccgtgctgtggtccatctgcagtggtgactctctctcactctctttatggggccactcccccacctaaattcctttgaggtgatttcaactggggtcagaatagagaggggagaaggaaaggtgtatgttcagctcatcagatttaactggaagctctcaaggctactttaaaaatcataaaagccattcccaataagcttgtttgttttaaaggaaatctcctttccaaatcactgtagatagtaaacagaagaagttgaaaaaaccaaataaaaacaggaaatatgatgaaagaatgtttcgatgtaacaattagtaaaagaatttgagctaccttgttaaatggcaaagtctatttattatgttgttaaagacaactgaaacaaatggcatttaaaaactccagatgagatgataaggcaaagcaatgccagatgaattcatcaagataaaaagcagtatggcaatgtttttatcaaagtagaattcaagtcatgaagcattcaacaggaagattattttatattgataacaggtacaggctatgaggggaaagctttgcaaagcaacaacagcaaaacagaaagcaaaaactattagaaggaagattagctatggaagaaaaagaaggctgtagagaattttaacaattattatgtttcaatcaacaaagaacaaacaggataaatcttaaaaagtggtcttgttattgttacagaaagtgatcattctttacactacaagggaaaactcaaaatctacaaaagagaaatttcacagacaacaatctctactatatccatacgtggggaacagaacaaaaaaactaggtctagactagaagacagagagaaaccatgtcagaccagagcacattgatggctcacggtgagtgacccatggcctaaaggtgcctgtttagggcccaggagccactcacacaggcagagcagcttactccgtatgaaccaccaccagcacccctccctgcccggtgatgtcacccggtgggctgggctggaacaagtccagatgcctttgcctcaccttggaagggccacgaggagcttcctcctctatccccaagttctccacttacacacagcacctgacacgaaggttggcaagtttcccccgggccatgactgcacaatggctacccccagcctctgtggcctccgagagagggctcctagacagattccagccctatagggggagggaagcaacactgcagttgaccttgaagagatcactgtagggggctatagaagggattgtgacatttattgttctgaaaatgccatcaaagacagttgtaaagtctagtctcatacacacttggcaagacatagccaaaagaggtaaatttgaaattagaaaaaatatcagcagttattacccagagcttgaaattctgacctgttacacagtaggatattcaacctccatttcagcgtatttaggtacttattaggtagattgcaaaattactagaaaaaaaattcctagaggacatcttgaaaatgataaagtagcaggaaaattacaaagatataacttatttacaaagtccatagagaagcgccattggaaagcttcaagttgaagataatttcatgaaaaacgcacttaaaacaaaaatggaattataatttttctgaactttggatactcttcaaatttccggaggtaccactcatgatgctcttttgctctaccagataaaaaacaaaacgtgaagaaagcaaaagccgcgccttggacagaccagctggccagggcatagccacaccactccatgatttctccaaaatagttggctgcagttacgtattcaaataagcctccccttggtattttgtatccagtatctcctggttttctgagattccttaggatatgatctgaatggatgtttatcaacatgcccgttaaccacaagccaaaacctattagaaaacggggatctgttacccagtcatcagcatacactgcacaatggctcaagtatctgctttgcaaatagccgttacaggtacagaacataatcgccattgtacacgccaacagtggcataggctttcctcctcgcatcagaaatgggtaaattaagcaccgatgcccgtagtggacgaggaacatggccaggaggatgcagttgggcgcgctgcggagacgcggggcggactcgctggcgtactggtagagcggcagggccagcgagggcagctcctgcaccacccaggcggcccgcgccggcactcggagcctgtggctgggcagcgcgtggcggccgtacactgagttcgtctgacgattgcgcgcgaagaccgcgcagcccacggcgcactgcaggtaggcgagcgcggccagcaggcgctcctccgccacccccgtcgccgttgccatcgccagggctgggcagcgtgctccatgccccagaggccgcggcgggcaacatatagggcggcggcgcgggggcaggaggggcggctaccggaggggcggctaccggagtcccgcactgccgggactctgcagaaagg

SEQ ID NO: 9596 - RNA, 4786 nt, Homo sapiens
  source 1..4786: mol_type = other RNA
atacccatagcttagctcccacatatcaatgagaacataggttgtttggttttccattcctgagttacttaacttagaataatagtttccaacaataaaaacaaagataaatagatgggacttaattaaactaaagagcttttgcatggtaaaagcaacagtcagcagagtaaacagacaacgcacagagtgggagaaaatcttcacaatctatacatcagacaaaggactaatatccagaatctacaacaaactcaaacaaatcagtaagaaaaaaacaaacaatcccatcaaaaagtgggttaaggacatgaatagacaattctcaaaagaagatatacaaatggccaacaaagtatgaaaaaatgctcaacatcactaatgatcagggaaatgcaaataaaaactacagtgcgatacccccttactcctgcaagaacggccataaccaaaaaaatcaaaaaacagtagatgttggcatgcatgcggcaatcatggaacacttccacactgctggtgggaatgtaaactattagagccaccatggaaaacagtgtggaaattccttagaactaaaagtagaactaccatttgatccagcaatcccattactgggtatctacccagaggaaaagaagtcattattcaaaaaaagatacttgcacgcacatgtttatagcagcacaattcacaactgcaaaatcgtggaaccaacccaaatgcccatcagtcaacaagtggtatatatatatatacaatggaatactactcagccataaaaaggaatcaattagcagtatttgcaatgatctggttgatcaatatcttaagaaaggtggttaagctttggttacagcaatggccgatagagaagattatggctgtatcagacacaagtgagggtcccttcccttttccttgcttttattcttgttatttttttctacctaacattattttagctacttacttgtttcttacctgtcactccacctgggccaggactgttttttctacccatccgtcctcagcacccactgctgtgcttgatatacagtaagtgcttggcaaatgttgttgaatgcacaaatgcatgcaccgctggccttggagactaaggaggagatgggtacaactattgttctctgcctcattggattttagctttggtcatgatagcagttggctgtggtcttcctacagataacagcagacagggtctggacggaaggagagaaatgggcttttgggttccaagttctgtcagtgttgggtgactgaagtcgtgcacagaggcctctctgagggagaagccatggccatgccaccccctggcttccctgcagcttgaggcaggaggtaaccagccattatggggcaggatccctataggccaaaatgtggagactttatttttttcctgggatgccaacacctagttctctggttttccccacttagttaatttttgtgttaggaaaggccacctcctcagcctaccttctcttccccggcaatgggcacatggctcatttctgggctctctgtgctctccctggagagtgggggtgcagaggacactgctttctgctgcaggcgccatgtttagttggtctcactttgagatgctcatttccctctgccttctgtcagcccagatgtgaggacccagggtctccgcagggtgtgcactgtcatggcctctctgctctgccacatcaggcccatctccacccgtgctgtggtccatctgcagtggtgactctctctcactctctttatggggccactcccccacctaaattcctttgaggtgatttcaactggggtcagaatagagaggggagaaggaaaggtgtatgttcagctcatcagatttaactggaagctctcaaggctactttaaaaatcataaaagccattcccaataagcttgtttgttttaaaggaaatctcctttccaaatcactgtagatagtaaacagaagaagttgaaaaaaccaaataaaaacaggaaatatgatgaaagaatgtttcgatgtaacaattagtaaaagaatttgagctaccttgttaaatggcaaagtctatttattatgttgttaaagacaactgaaacaaatggcatttaaaaactccagatgagatgataaggcaaagcaatgccagatgaattcatcaagataaaaagcagtatggcaatgtttttatcaaagtagaattcaagtcatgaagcattcaacaggaagattattttatattgataacaggtacaggctatgaggggaaagctttgcaaagcaacaacagcaaaacagaaagcaaaaactattagaaggaagattagctatggaagaaaaagaaggctgtagagaattttaacaattattatgtttcaatcaacaaagaacaaacaggataaatcttaaaaagtggtcttgttattgttacagaaagtgatcattctttacactacaagggaaaactcaaaatctacaaaagagaaatttcacagacaacaatctctactatatccatacgtggggaacagaacaaaaaaactaggtctagactagaagacagagagaaaccatgtcagaccagagcacattgatggctcacggtgagtgacccatggcctaaaggtgcctgtttagggcccaggagccactcacacaggcagagcagcttactccgtatgaaccaccaccagcacccctccctgcccggtgatgtcacccggtgggctgggctggaacaagtccagatgcctttgcctcaccttggaagggccacgaggagcttcctcctctatccccaagttctccacttacacacagcacctgacacgaaggttggcaagtttcccccgggccatgactgcacaatggctacccccagcctctgtggcctccgagagagggctcctagacagattccagccctatagggggagggaagcaacactgcagttgaccttgaagagatcactgtagggggctatagaagggattgtgacatttattgttctgaaaatgccatcaaagacagttgtaaagtctagtctcatacacacttggcaagacatagccaaaagaggtaaatttgaaattagaaaaaatatcagcagttattacccagagcttgaaattctgacctgttacacagtaggatattcaacctccatttcagcgtatttaggtacttattaggtagattgcaaaattactagaaaaaaaattcctagaggacatcttgaaaatgataaagtagcaggaaaattacaaagatataacttatttacaaagtccatagagaagcgccattggaaagcttcaagttgaagataatttcatgaaaaacgcacttaaaacaaaaatggaattataatttttctgaactttggatactcttcaaatttccggaggtaccactcatgatgctcttttgctctaccagataaaaaacaaaacgtgaagaaagcaaaagccgcgccttggacagaccagctggccagggcatagccacaccactccatgatttctccaaaatagttggctgcagttacgtattcaaataagcctccccttggtattttgtatccagtatctcctggttttctgagattccttaggatatgatctgaatggatgtttatcaacatgcccgttaaccacaagccaaaacctattagaaaacggggatctgttacccagtcatcagcatacactgcacaatggctcaagtatctgctttgcaaatagccgttacaggtacagaacataatcgccattgtacacgccaacagtggcataggctttcctcctcgcatcagaaatgggtaaattaagcaccttaatagagcaggaaaaactgtaaagcttgttatttgtttccattctgaccatgtgcgccagggtaaagtcataattagtcattagttatggttatgaacgtcgacagtaatcacataatagtagtgtcatgctggctgtgcatcctcaagccactctctccccagcactcccacttaactcctggggaagacattcacatgagtcaaaagcagcctccaaggttctcatctcattcaggccaggacccctaggaagacttcatactgatttacagcaaagcacgtgttggccagtaagtgtgcattcagatgttgtgtcatcagtgaggtgggtattctcctggaagctgcagtgttgccaagcaatgaataagaacaacgaatcccagcaatttctctctgcgtcttggaatcatgattcagatccgggcagacaatgggtaccatgggctggcatttgggatgtaggcacactgcaagtgcttgcataccaacatttccgatgcccgtagtggacgaggaacatggccaggaggatgcagttgggcgcgctgcggagacgcggggcggactcgctggcgtactggtagagcggcagggccagcgagggcagctcctgcaccacccaggcggcccgcgccggcactcggagcctgtggctgggcagcgcgtggcggccgtacactgagttcgtctgacgattgcgcgcgaagaccgcgcagcccacggcgcactgcaggtaggcgagcgcggccagcaggcgctcctccgccacccccgtcgccgttgccatcgccagggctgggcagcgtgctccatgccccagaggccgcggcgggcaacatatagggcggcggcgcgggggcaggaggggcggctaccggaggggcggctaccggagtcccgcactgccgggactctgcagaaagg

SEQ ID NO: 9597 - RNA, 640 nt, Homo sapiens
  source 1..640: mol_type = other RNA
atacccatagcttagctcccacttaaaagtgagaacatatggtgtttggttttctatttctgagttacttcacttagaataatggtctccagctccatccaagttgatttataatactgaatccattaattcccaggtttctgctttctcagcttcttgaagatagattcaatggtgccactgcaaacaggtgactaccaaaacagcaagatacacaaaagaaacatctccttttagtgtgtccatgtgcgtaatttttcctcgttgtgagacaagaacccagatttagctgagctgaggagcaaaaaatcctgcatcaatagaacagatattattatttatatttcacagatcagaaaactaaggcccagagaatttaagtaatttctgtacctagggtcacaatgtatcagttcagggctcacattccctaaagtgccttcagatagtgcctaaatcacaaatcaaaacttctgtcattctcattctttgcattcctttgaaagaaagcaggaagaaaatacctctttcaaattgaggaagctcagcggtcttctgtttacagtcatccaagatgggcaacataaaactctagttgtagtcatgcacataatggtctctgtaaacagtgcttcctgga

SEQ ID NO: 9598 - RNA, 149 nt, Homo sapiens
  source 1..149: mol_type = other RNA
atacccatagcttagctcccacttatgagaacatatgatgtttgctttccattcctgaattcgcttagaatagtttccaataccatccaggttgctgtgtatgccattaattcattcctttttatggctgagtagtattccatggtgtg

SEQ ID NO: 9599 - RNA, 4443 nt, Homo sapiens
  source 1..4443: mol_type = other RNA
atactgtgaatttcactgtcacaaattcaaataaagtgagagtggaattcacagtatttaaggaatcaatccttgctgcttctgtttatgaagccgagcttcagttttcttgctctgacaatggacacagtgattacctcaagggttgctgtaggagttagatgagatatctataatgtaggaaaggtgtttactacaatgtaactcatggataggggcctatattggttttccattgctgtgtaacaaatttccataaacttagtggcttaaaacaacagacatttattatctttcatttctgtcagaggtccaggcaactgagtggttgatatctctgttcagggtctcacgaggctgaaatcaaggtgtcagttagctgcattcccctctagagacttgactagggaaggattcttttccaaattccttcaagttgttggtagaagtgtttcttgctagcttcaattagggatggatctcagcaactagtgaccactctcaagtctttattatatggccccttttatactcaaaaccagcaacagagaattccccctcacatcaaatccctctcacactttcaatctctatgactcagaaacgggctcacctggctaggtcagacccaccagaatattctccattttggctagctcacagtcgcctgatgagcaatgtaatcatagcagtggtatcatacacacaggtctgcctgcactcaaaggagagtgattatcaaggaatgcacaccaggggcggcaggaatctggcagctatcttagaattctgcctgccaccatttccattaagtgattgttgttgtttgttactgaggcatagatgaagtagcacttatgcaggaaaaaaaccactagtcaatcagaatttcaagttgtatgatgaggtattccatagaaattaaacatgcgtataacagattctcataggtcaggacacatgaaaaatttaaggaaaggatgaggactccttaatttagagggacttctgaaaggtgacttaatgatgacccaacactatatgtgaaatcatgtttggcttcaaaagcactgtgggcagaaaaggagaaaacgtttaatctagagtacacagttatggcattatctggagggaaggataaagctacaaagattgttaaaactaaaatttgttgccaagggagccattcgagctctgtctggagatcttctaaatgagagtaaattattctgtacttgaggtggtttgggcactgtcctccctgaagccaatgtagagataaagtgttgttttcactccttctagtcctgtgattctgcgtctaaggaggcaaaccacctattgaatcagtgctcaccacaggctccattgcagcattgaactgtgtctgtgagaaagaataaggttaagtcaggattccttgattaagacgagttaatataaacactgaaaatccagtgtgctgccagcatagcttttggcagcatcaacacagagaagaaagagctgtaacagaataacagcaaaataacttcgggtccttccttctcctccacccacaaaatcccatttggtgatatgagaatctaaattgctcagtgcttggatgtttggctgtcacatgtcattgttgtgttgaaccttcccaggcatgtacagagctcactgctcaggagattaatgttcaaaagccaaaatgcttgaccaaacttgaaatctatttgtggaatttactgtttcatcattgaaccatgaaaaaataaattcagcaaatatagtcctaatactccagctcatcatgaaatgtctcttaatttcttgacgtgtccatgagttagagacagctgagaaaggtttcattatctttgtctacttacatacattctttctcatttctttttctttttaaaatctaaggctttttttacttgagaaaggagttgttccgattactgtcagtttctctggctgatgtgattttctcatcagaagccttgaacccttctccttttaacttgatagcaaagagaaatcatgatagcttcttttgacatcactttacacaaaaacaaacaaaacaaaacaaaattatcataaactggtagaacaagaagacagcatgtagggaacaaaacaaccatgttcttgattctaatgaggtacatgatttactcctaccatggaaaattcaaatatctacccttgaacttcaacaagcatttatgacttgttgatctacttatagaactaaatgattattttgcaaaacatcatctctgtctttaagtactccctacagaagaaagaaatggaacattagtgtaaacatgatggtcactaagaacttgtggacactgaagaaaggctatggataaatgatccaacaataagagaaagcttctgagtatgcctcagaccagtgactgactgggttttctgggaatatattttttggacaatgggtccaggaagacaataataaatattggaaaaacttcctacagtctataaaatcccttttatttagataatctcactgggaggaaggtaaggagagggatatttattgagagtccgtgacagagagatacactgtgaggtacctttcaggttccatctcattaatttcttaaattgactctaaagaggaatgttacctcaattttatagatgatctccaaaatcctcaaagcttttaagtaacttgtcactctgcataagaatttgcctccaaacttagggattttaaagaactttgtttttcttttttctatgtcacccagagtatttggtcaggaaaagaacttgcagttctcactcatagtcaatttgttggtagtagccactgggtcttcagtccttggaagtctagactgggctggactttcaagatggttcacttaatgactggcagatgtgactggctgtcaactgggacctctcaggggactgttgaccagaatacctacatgtagcctctatagcatggtggtcttaagatagccctacttcttatatgatggacagcctctccagataaagtgttgcacaagatcaagtagaaatgacctgacccttctgagcagcatcaggaattacacagcatcgcttcctccatactctatcggttgaagtaattagaagcccaccaagacttcagggaaagggacataaaagctatcttttgatgaaaggaatgtcaaaatattttggggccatgttttaaaattaccatacttgctcaaaatacaacagcaagtaagtgtccactaaaataaaatacaactcataatgtgtgatggacttttttaaaatttgtaaatggtggaaattgacatcagtgagattaaggctagaagaacgtatacgtttgtaaatcaaatcacaggaaagggaagatgaatatggctttagtcacgtgtggttctaggcaccactgcagaagctttttccatcaactgcatttgattcgctctgtatgttggctgcattttatctattgtagaccactattttcataatgctccagcaacagcaaatgtcatctaaaggaaggaactcctgctccttggttcaaatttgacatactgcagagaacaattttgatacctagtttttgtcacatacaatcacctgttcagtccttatagcagatcctatttgagtcacgtggttagaacaatcctcggtattatagaagattccaaggtgaaaggaatagaaggaaaaatgggtaaaatatggccactctatagaaatcaagagaatttacagtgaatagtgaactaactaccatctctttttgctaagaaacgctttgggacaattttgtaaattttacaaaggaaggaattagtctttatctctcagcaaaccttttgttgaccagaggatccttggaaaaccaaatgaggggctatgtgatttatctgataatgagctagaaatcagagcatatacacacatcttcatttatgtaccacttttcaagtatattcacatgattatttcatttacacacaatagctaagtgttataggacaagttttatcttcattttatagctaagaaatctgagacccagaaagtttaagtgacttaatcccagttacatagggaataaatagcagagctaggacttcaactcagattcctcctcttagaccagtatacttttcaccgcgccacaggttcgcctaatgtaaaacttaagtttcattgatgacatgatacatgggtaaaggttttctctactggaggttccaaccacttgactatctcatcttagagtagctgcctgacaaagcattttggcttctatagagtaaattaaacatgcccttttatgaatgaaattcataaaagtaaatttcctttgccaagattatccttcttaaacatgacatccccttccgtagacaccacttatggtctcccattaca

SEQ ID NO: 9600 - RNA, 63 nt, Homo sapiens
  source 1..63: mol_type = other RNA
atagcagcataagcctgtctcaaaataattctgcagtgagacaggttcatgctgctatcgttc

SEQ ID NO: 9601 - RNA, 86 nt, Homo sapiens
  source 1..86: mol_type = other RNA
atagcagcatgaacctgtctcactgcagaattattttgagacaggcttatgctgctatccttcaaaagaacacatccacccagcta

SEQ ID NO: 9602 - RNA, 60 nt, Homo sapiens
  source 1..60: mol_type = other RNA
atataatacaacctgctaagtgctaggacacttagcaggttgtattatatccatccgagt

SEQ ID NO: 9603 - RNA, 60 nt, Homo sapiens
  source 1..60: mol_type = other RNA
atataatacaacctgctaagtgtcctagcacttagcaggttgtattatcattgtccgtgt

SEQ ID NO: 9604 - RNA, 68 nt, Homo sapiens
  source 1..68: mol_type = other RNA
atatgcctggctagctcctccacacgcatttgtggaggagctagccaggcatatgcggagacttgcca

SEQ ID NO: 9605 - RNA, 35 nt, Homo sapiens
  source 1..35: mol_type = other RNA
atattattagccacttctggatttcttccatatca

SEQ ID NO: 9606 - RNA, 80 nt, Homo sapiens
  source 1..80: mol_type = other RNA
atcaaggatcttaaactttgcctttgtagctctggcaaagtttaagatccttgatgttcctggaggactggtggatgaag

SEQ ID NO: 9607 - RNA, 2811 nt, Homo sapiens
  source 1..2811: mol_type = other RNA
atcacacaaaggcaacttttgtgtgtgaaaacaggaatgcatgttctcagttagggccagaggtttccaggcttgaaattgggacctttgccagggaactgccctcttctacccagtatttctctgtctcctagccgtatcatctcccctctctgcagaggcaaatctaactgccattagaatatggacgatggccaatcttagctaatttctgctgacaggtggcactattttggagaaaacagcagtcagattcctcccagaggtttatctaagggtccttgcaaaagggagccgttgtccgaggctccggttgcctgaccatttggagtttgatggcctctaagtgagaggaaaaaacaagttttataaggttaagtaggcatgggttaaacaagtgtattatacaagaaaataatctagtgccaaagatcacagaaataacaagtgaaaatactaaaaccattctgctttgagctgtttcaccctggtgaaagaaattaaaccttgtatagaagcggttcaactttagaagagagacaactgttcttgccacatctgtagcaattaacaagtgtaccctgggaattctggggtttatgggcttgcatggtgaccattaatgcttctgcctctttcttgtgtcccccatctctattgtaaaaggcaaagatggccactttcagttagacctctaaagtattatctggtcccagggcccatttctgcaacttcctcctgatatcaggggctgtctgagtaataaatttattcttcagaattagttgtcccttcactgaatcagaagatacgggggtatgctttaccaaggcccctcttagcctctccaagaaggcagtgggattttcattaaatccctggtctatcatagatagcttgctataatcaagaggcttggtcttagtcctacgtaatccctccatgatgcatacctgaaagtatctcctcttccagtctcccatttcaacactgggatccatcccatccagggtcatttactggtactgcttctcttccagtcggataaagtttgccccctttcctgacactatatgtgaaacaaagctcatccccaaatctctctgctacttgcagagcagcctgcttctcagtgttcatcaggatctgattcaaaagtaacacaatgtctctccaagagagttcaaatacctgggttaaattctggaaagcctctatctatctgtcagggtcatgtgaaaacttgccaaaaatcccccttaatgtactttaagtcctgtagggggaaggagacctgcaccttactggggccaaattcacctggcatctgttggaagaggaggagtgagactggggcttgtctagggtgaggatttctaggattaggcaagcgagagactgaagctggatagagaggttgaggtggacccagaggagcagagctggagggagctggcttctctgctgggagtgcctctgggatttgtttctttagttccctggaattgccctttgcagcctctcctgaaatgacaaagcaggagggctggatcaatcctacactgtcagcaaagatctagatttccctgcaaggtataaaaagcctgcacatgtggggcctcaggccattcgtcctcacgcctacagaaaatgtccagctgccagatggtatcacaatgaatggttccttcctgagaccaagccagtccttcataatttggccaaacctttgttccgagggctaggaggtgtttttcctccagattctgagggtcaaagcagactcagtggttcaggatacacaggctaggaggtgtttttcctccagattctgagggtcaaagccatctcagtggttcaggatacactccagaggagaataagctgggggtggtgaagagagctggttgcccattttgtggtactggtttaataggtttttccatcaagcctccaatataaacagtgttgggaagcaggggccgggcaaaatcaaaggcaaaatcagagttaacaaaccacaactctgctttcagtagaagatgagacaaaactggcctagagccttctgggaaatgctccttgatggtgttgtcaaatgtagactgcatgtcccattggctcctggagaaactaaagaacatcagaaaattcttcactcggccccagaagtccatgtgatcagtcagcaaggaagggaatactggaacataagacaaggggcttggtagcccaaaatccaaagagccgaatgtggtgggaagaatggccacaaatggtttcacaagcttctcagcaatcaggaaagaacagaaatcaaatgcttcaacaaataccagatcatagttctcattctttaaggaatccattatatcctttctgcttagcaaataactacattgagtcccaaatatttccattagctttacaagggcttcagattcttttctgccatccaatgctgtttctatgtagctatcaaaatgcttcttaattcttttttgatgatcttcaggtgaaaaccacctgataacttggtatgatttttcctcctctttaatatctgggatcaaaaactttccactctgatgaagcatagtcacattatgaccatgctcttgaagaatctgagacacccggtccaacagtaggtaatggcttccacacagccagtatttctcagttgtgggtctctgcagtgccttctttagtattcctgtaggtccagacagccaatatttggatatttgcctttatggatatgtggactcatgcctctttccagtggctctggtctaccatggtgggtat

SEQ ID NO: 9608 - RNA, 1455 nt, Homo sapiens
  source 1..1455: mol_type = other RNA
atcatacaaggacaatttcttttcgaaggcttattccagtttcgtgaggctagcatgaggtgtgtgcatttgccaggggcaaatttctattctcaattaacccatgcagcaaatgctacgcatctgctgagtccgtttagaagcatttgcggtggacgatggaggggcccgactcgtcgtactcctgcttgctaatccacatctgctggaaggtggacagtgaggccaggatggagccaccgatccacaccgagtacttgcgctctgggggtgcgatgatcttgatcttcatggtgctgggcgccagggcggtgatctccttctgcatcctgtcggcaatgcccgggtacatggtggtgccgcccgacagcaccgtgttggcgtacaggtctttgcggatgtccacgtcacacttcatgatggagttgaaggtggtctcgtggatgccgcaagattccatacccaggaaggaaggctggaacagcgcctccggacaccggaaccgctcattgccaatggtgatgacctggccatcgggcagctcgtagctcttctccagagaagaggaggatgcggcggtggccatctcctgctcgaagtccagggcgacgtagcacagcttctccttgatgtcgcgcacgatttcccgctcggccgtggtggtgaagctgtagcctcgctcagtgaggatcttcatgaggtagtcggtcaggtcccggccagccaggtccagacgcaggatggcgtgggggagggcgtagccctcgtagatgggcaccgtgtgggtgaccccgtctccagagtccatgacaatgccagtggtgcgcccagaggcgtagagggacagcacggcctggatggccacgtacatggccggggtgttgaaggtctcaaacataatctgagtcatcttctctctgttggccttggggttcaggggggcctcggtcagcagcactgggtgctcctccggggccacgcgcagctcgttgtagaaggtgtggtgccagatcttctccatgtcgtcccagttggtgacgatgccatgctcaatggggtacttcagggtcaggatgccacgcttgctctgggcctcgtcgcccacgtaggagtccttctggcccatgcccaccatgacgccctggtgtctggggcgcccgacgatggaaggaaacacggctcggggagcgtcgtccccagcaaaaccagctttgcacatgccggagccattgtcaatgaccagcgcggcgatctcttcttccattgcgaccccgccttttgttcccggggaaggcgcgacgaggcctcggcagctggaagcggggccagccggggtcggggggcgcaggcctgcgacgtccagctcaggccccggggcggggcgctcaccggcagagaaacgcgacggcggagcggcggaagaacagagtgcgagagctggcagcggcgactgag

SEQ ID NO: 9609 - RNA, 1336 nt, Homo sapiens
  source 1..1336: mol_type = other RNA
atcatacaaggacaatttcttttcgaaggcttattccagtttcgtgaggctagcatgaggtgtgtgcatttgccaggggcaaatttctattctcaattaacccatgcagcaaatgctacgcatctgctgagtccgtttagaagcatttgcggtggacgatggaggggcccgactcgtcgtactcctgcttgctaatccacatctgctggaaggtggacagtgaggccaggatggagccaccgatccacaccgagtacttgcgctctgggggtgcgatgatcttgatcttcatggtgctgggcgccagggcggtgatctccttctgcatcctgtcggcaatgcccgggtacatggtggtgccgcccgacagcaccgtgttggcgtacaggtctttgcggatgtccacgtcacacttcatgatggagttgaaggtggtctcgtggatgccgcaagattccatacccaggaaggaaggctggaacagcgcctccggacaccggaaccgctcattgccaatggtgatgacctggccatcgggcagctcgtagctcttctccagagaagaggaggatgcggcggtggccatctcctgctcgaagtccagggcgacgtagcacagcttctccttgatgtcgcgcacgatttcccgctcggccgtggtggtgaagctgtagcctcgctcagtgaggatcttcatgaggtagtcggtcaggtcccggccagccaggtccagacgcaggatggcgtgggggagggcgtagccctcgtagatgggcaccgtgtgggtgaccccgtctccagagtccatgacaatgccagtggtgcgcccagaggcgtagagggacagcacggcctggatggccacgtacatggccggggtgttgaaggtctcaaacataatctgagtcatcttctctctgttggccttggggttcaggggggcctcggtcagcagcactgggtgctcctccggggccacgcgcagctcgttgtagaaggtgtggtgccagatcttctccatgtcgtcccagttggtgacgatgccatgctcaatggggtacttcagggtcaggatgccacgcttgctctgggcctcgtcgcccacgtaggagtccttctggcccatgcccaccatgacgccctggtgtctggggcgcccgacgatggaaggaaacacggctcggggagcgtcgtccccagcaaaaccagctttgcacatgccggagccattgtcaatgaccagcgcggcgatctcttcttccattgcgaccggcagagaaacgcgacggcggagcggcggaagaacagagtgcgagagctggcagcggcgactgag

SEQ ID NO: 9610 - RNA, 6785 nt, Homo sapiens
  source 1..6785: mol_type = other RNA
atcatacaaggacaatttcttttcttttttttttttttttttgagacagtcttactcggtcacccaggctggagtgcagtggcgcaacctcggctcactgcaacctctgcctcctgggttcaagcgattctcctgcctcagcctccggaagagctgagattacaggcgaccacgactgcctaatttttgtattttagtagagacggggtttcaccatgttggtcagggtggtctcaaactcttgacctcaggtgatccgtcccccttggcctcccagagtgctgggagtacaggcgtgagccactgcgcccggccccaaaggacaatttcttgagacccccacacaccttcagaaccacacattctgttcatgttaaaaacaagaaattaacaacctctaaagctaaggacaatgattctgtaaagtgcaagaatggttcattgtttccgcttttgtggatttcatgttaagaatactttaaaagaaagggtgggcgggagtaaaccaggaccccagtcatatatttgatcaagaaatgacccgtatggcaaaggtgagacgtggaccagccctcaggtgtctccaactctgtgcacaccactgaggtaggagctctagaagaaacgcagaccctctcaggggggttaaggtttcctcttggcaaatgagctgggggcctgagacagtcatacccacgggctgcatgcaactttgcatgcaacttcacgaaattctagagctgtatcacatcagcgatggagaagggcaagatccaagacaaagccacatgaggcgaggtcctggtgctgccatttgttgtccagcacaaatcaaggggccggaggaaagggatgaggtggaaaaccccggcaggcattctacaaaacagttattagcaaattgtatcaaaaagtatcaaaacatttcaaaaaactctaaaaactgccaggcttggcagatgcgcaggacagggtctccaagtgcccgtggcgctgccctatactccaggcatttatcctagaggccaggatgccaccccctcccctcccctcctgggcactcagaatccacggagacaccaggaggtctaaacctcatctgcagctgcccctccaggtttgggaccagtggacggggttccaaccacgggctctgacagccacaaggcccatgagatgctgctgcaccatggaggaccagggtgaaggatgaaggtcagtgactctacagggggtggtggggggtgtggcaggggtcccctcacttcccacattgctgcaagtcactgaacgatcacttggcttaggggccgaggtacactgaaccacaggtgaacacaactgagctcacaaagtaggcccctggacctcagaggatggaccccacttcccctcagcatctggatgcccacctcaaaggtgaacaccccttagggtgagtttctgggtctccatgaagtcaccttatcatgagtgagggcactcaatataaatacacacgtgtggtcctgctcagagccaggtctgaagtcccacttgatagcctcaataaaatggcagaacaataaaaataccaattgcgtgctaaccacagttgataaaataatctctgtgcatttaaaacagcaggaagtttgctataagtaacaagggttcatcagctttctactccctcccttctattattataatacatctatgtcttaagcaaacagctttccaacttgggtgaggaccaaaccccaaacttacaactaatatgaagttacaactctaattctttagaaatgagagaagtccaaacctcaatagaagcctgccatgcttattttgaaatgttaaaaaaaaaaaaagatccaggtgtcttcaaaattcaagcagaatagcttgaaacactgaaagtttaacatgatgacatgtgtggctgtttccctctcaaaatggcagcctgcaagcacctgtgccttcatcactctagtttaaaaccccacattcgtgactgtgcggttcaaatggccactgcataagcacagcccaaactctgcccatctgagttaaaaaacattttattcttttgagacagggtctcactccgtcacccaggttagagtgcagtggtgtggtcatagctcactgcagcctcaacctcccaggctcaggtgattctcccacctcagcctcctaagcagctgggactactgcatgccccaccatccctggctaatcttttgtaatttttttgtagagatggggttttgccatgttgcccaggcatggtctcttccattttcagttccattttcatgcacagtagggtgaattttcaacttaaaaagacaagtaacaaaaacctggcccgggcaccaccactgggtgcccttgtgcccatccactgaccccaacaagctcaaaaacctttcttgtcacagtgtagccaccatcaaatattagaagttgacccacaagatgaaacttgtttatcctccctttaaaagggtggtcccaaccttagtaatattagggtcaaagccatgtcaattacaaaccaccttcatagtatcaggagagacaccacaaaatatgaagcgcaggacgtcgtatgtaactcatgaggcacaagaaaatcagaatagaggccagaagctcacacatttccagggacaagtcccagaagcaaaacataaaagagctggcttaggctgaaaaccaatggctctcctctctccaaggtcaaagctatcccactccccaaatcactcacagagtctttctatgtgctctccccaacttgccccgagattcaggccaaacaactgcccgtttgttcatgacccaggctgagatggggagaacagcccacgtacaccctaccctgccttctgaggggtctacaagcaataaaacctttcccgaataggaagggggtaagctatcccaaagttggcagaagttctgcaaaacatgttttgtgggggtctgggactaggtatgagacaaacgacttttaggctcaaagaagtttggaaatgctgggttgagacttctcggaacctttcatacaccggaatgctgcagagctccaagcagagtttccagccttttggtctgtttgtttgtatgcctcgcagaacctctcaacagtttgtaagcctccagggacttcacatgcaaataactagctagctgaacatgcagactgccctcctcactaaccacagagggcagtaagttggctattgaagctttcagtccccaaaatgctctcatctcttctggatggctacataaacagaccagtgagaaccacagtaaaccctgaagggaagggaaaggaggggcagcaaagaagcagaagaaatggaaattaaagttaactaagatttttttcctagtctaatatcaatcttaacacattgatcctcatccactcgagcagctgagagccctcttaaagggcaagtgacatcgagacctgctctcggaactgtctgcaggaagactggtgttagactaggattgaagatgaagcacatcttgaagtttactgatctctgccatcggatgctgggtgaggtacagctcattcatgccttccttggctcatgcttaaaacccatcacactcctatcctcccatagttctgcacgtttctcatccactcgggcagctaagagccctcttaaagggcaagcgaccctgacacctgctttaggaactgtttgcaggagtcagtgcaggccagctccacatcctgaaggggatgccatccgggtacgaacagctcagaggctgaatggccctatcacccgggaggagcctggagggtattccatctaatcctgtggctaagcggggtggatgagggaacacacggacttgttcgagaatttgcccagcagcacgaaactacttagaagcagaaaactggggcaggacctggcgtgggagttagggagccctccactgccttctcagggatccacatgtgctcctctgtgcaggaactttcaacagcgcctcaagatagagtcacagagaacgatggcaaattccatagcactcactttttctttcctgagaaataaacagatttgggagctcagtacatcagtaatataaaagacagtgggttcagaaaaaaaaaaaaggaaaaaaatgcacaaattacaaaaaaatatgtataaagagcttcataccttttttcgtttttggttacctgtaacgttttagaattcaagaaggtttccaatgaggaaagacggaattattcagaaacagcgttcacctgatacggagaacagctccccagcgggaagtcatcatgtctcatctgacagtctagcgagctgcgtggcccctggtcactcactcactcaccctcatgggtggtctctgtgcactcatttataaaacaaacacactggaccttgccagtgattcccagatgtgactaatacccagaattccaagaactagttaaaatacagcttctgggcaccacctcctccccgttcctggtggttttggattccataattctgagcggggctcacgcatctgtattcttaaaagttcagccaggtttggggaggcttggactaggtggcctaagagaaccctttgaggcccaagcttcactacagaaatttctgtgttacccacgtgccagctactctcagggggacagtcagcaaggacccatgaggaatcataacacggggcaaagacctgtgaagatacaaggggttgctcactgcctgggcccagggttagttattcaagcaagatatgtaaagttacagatagtatttaattggttactgtgatatcatagaaataccaagaatcataaaagtaaaaaaagctgctaagttgtacataatgtttccggaatactaagaagttgctgctggtctacagagccctgggaggtgacggtgaggatggtcccaagaggcgcagctagggtcactggccccggtcctggtgcctcttgcctttgcctttcttcttcttgtcctctggccgtggctccagggcgcagacacaggcggacccgccagcgatggccttgggcaggtcgacgcccctgctccacttgtcggcctcgcggtcgtacacctgcacggtcttggagaaggcagtgttctcccagctgtagccgcccaggatgtagatgcggccctcccacactgccacgcccgactcgctgttggcgtgcagcagcggcgccacgcgggtccactggttgcactgcgggctgtaggcctccacgcccagcacgtcgaagcgctccatggactcgatgttgtcatcgctgcccccgatggagtagatgctgtcacccaggctgcacatgctgtgccagccgcgcgccgtggtcatgggccgccgctcctcccacacgtctgtccggtggtcgtagcatagcaggttcttgcggtaggggccaatttggtagtcgtggccccccgagatgtacacgaagtctttgtagatggtgcccgcgtggccgtacgtgaacctataaagaagattggaggccgcatcccctccgttgtcccgtgagaagctgccgccggcgatgaagatgaagccccccagcaccgcgacacagtggtggctccgccgggcgggcagcggcgtctctttgacccactgctcgctcttggcgtccaggtagcaggtgtcgtcactgagctccagacaccgctcggagacctcgccgcccacaaacagcaggcgctcctggttggtgcgcagcgccgtgcgcttggtctgcatgacgggctgggccgccaggttgttgtggtagcgcacggcctcctcgatgaagccctcgcagttggcctccttgggcagcagcgagcacacggccggcttgacgcggtgcagcaggtcgttcttggggatgagcgggaagtggatgttctccagcacctggcgggcgtgggcctcgcgctcgggctgctgcgtcagccactgcagggcggcctgcaggaggtcgtgctcacactcccgctgcacctcgctgctgctcaggtagacacacagcttctgcatggagacgttctgcaggaagtcgggcgtaaaggacagcgtgccgaagtggttcaggatgaagccatcgatgaaggcatcaagccgcttgaggctgtagatggaggccagctcctgcaggtacaggtagttgtcctcgctcacctcctgctccaggtactcacagcagaagtctaccaccgtccagatctgcagcaggtgagccgtctccaggacgtagtcaatgttgccgccatccagcaccagctccccgccgtacaggaagtccaccacggccttgagcccaatgtaggaggcgccgatcagctccacctccttctggaaagcttcccgcatgccgatggtgaacatggagttgaagtagtcgctgcacacggccagcaggttgcgatgggctggcacacgctgctcatcggccaccaggacgacgtcgcagaagagcccgcggagacgctgctcgttcagccgctgcagcaccgtgcttgagtggtcggcccagcggtatacctttgatgattcgctgatcttgtatggccgagacactcgcgtctgcctgcttccctccatcattaaagagatttcagccctggcaggacgcgctacggacgcggcggggacagccccggcggcggggccgggcggtcggggcggcggggcccgggttcaggagacccccggccagcccgctgcgcagccatggctccgccaggaagtgcgaggccgag

SEQ ID NO: 9611 - RNA, 6937 nt, Homo sapiens
  source 1..6937: mol_type = other RNA
atcatacaaggacaatttcttttcttttttttttttttttttgagacagtcttactcggtcacccaggctggagtgcagtggcgcaacctcggctcactgcaacctctgcctcctgggttcaagcgattctcctgcctcagcctccggaagagctgagattacaggcgaccacgactgcctaatttttgtattttagtagagacggggtttcaccatgttggtcagggtggtctcaaactcttgacctcaggtgatccgtcccccttggcctcccagagtgctgggagtacaggcgtgagccactgcgcccggccccaaaggacaatttcttgagacccccacacaccttcagaaccacacattctgttcatgttaaaaacaagaaattaacaacctctaaagctaaggacaatgattctgtaaagtgcaagaatggttcattgtttccgcttttgtggatttcatgttaagaatactttaaaagaaagggtgggcgggagtaaaccaggaccccagtcatatatttgatcaagaaatgacccgtatggcaaaggtgagacgtggaccagccctcaggtgtctccaactctgtgcacaccactgaggtaggagctctagaagaaacgcagaccctctcaggggggttaaggtttcctcttggcaaatgagctgggggcctgagacagtcatacccacgggctgcatgcaactttgcatgcaacttcacgaaattctagagctgtatcacatcagcgatggagaagggcaagatccaagacaaagccacatgaggcgaggtcctggtgctgccatttgttgtccagcacaaatcaaggggccggaggaaagggatgaggtggaaaaccccggcaggcattctacaaaacagttattagcaaattgtatcaaaaagtatcaaaacatttcaaaaaactctaaaaactgccaggcttggcagatgcgcaggacagggtctccaagtgcccgtggcgctgccctatactccaggcatttatcctagaggccaggatgccaccccctcccctcccctcctgggcactcagaatccacggagacaccaggaggtctaaacctcatctgcagctgcccctccaggtttgggaccagtggacggggttccaaccacgggctctgacagccacaaggcccatgagatgctgctgcaccatggaggaccagggtgaaggatgaaggtcagtgactctacagggggtggtggggggtgtggcaggggtcccctcacttcccacattgctgcaagtcactgaacgatcacttggcttaggggccgaggtacactgaaccacaggtgaacacaactgagctcacaaagtaggcccctggacctcagaggatggaccccacttcccctcagcatctggatgcccacctcaaaggtgaacaccccttagggtgagtttctgggtctccatgaagtcaccttatcatgagtgagggcactcaatataaatacacacgtgtggtcctgctcagagccaggtctgaagtcccacttgatagcctcaataaaatggcagaacaataaaaataccaattgcgtgctaaccacagttgataaaataatctctgtgcatttaaaacagcaggaagtttgctataagtaacaagggttcatcagctttctactccctcccttctattattataatacatctatgtcttaagcaaacagctttccaacttgggtgaggaccaaaccccaaacttacaactaatatgaagttacaactctaattctttagaaatgagagaagtccaaacctcaatagaagcctgccatgcttattttgaaatgttaaaaaaaaaaaaagatccaggtgtcttcaaaattcaagcagaatagcttgaaacactgaaagtttaacatgatgacatgtgtggctgtttccctctcaaaatggcagcctgcaagcacctgtgccttcatcactctagtttaaaaccccacattcgtgactgtgcggttcaaatggccactgcataagcacagcccaaactctgcccatctgagttaaaaaacattttattcttttgagacagggtctcactccgtcacccaggttagagtgcagtggtgtggtcatagctcactgcagcctcaacctcccaggctcaggtgattctcccacctcagcctcctaagcagctgggactactgcatgccccaccatccctggctaatcttttgtaatttttttgtagagatggggttttgccatgttgcccaggcatggtctcttccattttcagttccattttcatgcacagtagggtgaattttcaacttaaaaagacaagtaacaaaaacctggcccgggcaccaccactgggtgcccttgtgcccatccactgaccccaacaagctcaaaaacctttcttgtcacagtgtagccaccatcaaatattagaagttgacccacaagatgaaacttgtttatcctccctttaaaagggtggtcccaaccttagtaatattagggtcaaagccatgtcaattacaaaccaccttcatagtatcaggagagacaccacaaaatatgaagcgcaggacgtcgtatgtaactcatgaggcacaagaaaatcagaatagaggccagaagctcacacatttccagggacaagtcccagaagcaaaacataaaagagctggcttaggctgaaaaccaatggctctcctctctccaaggtcaaagctatcccactccccaaatcactcacagagtctttctatgtgctctccccaacttgccccgagattcaggccaaacaactgcccgtttgttcatgacccaggctgagatggggagaacagcccacgtacaccctaccctgccttctgaggggtctacaagcaataaaacctttcccgaataggaagggggtaagctatcccaaagttggcagaagttctgcaaaacatgttttgtgggggtctgggactaggtatgagacaaacgacttttaggctcaaagaagtttggaaatgctgggttgagacttctcggaacctttcatacaccggaatgctgcagagctccaagcagagtttccagccttttggtctgtttgtttgtatgcctcgcagaacctctcaacagtttgtaagcctccagggacttcacatgcaaataactagctagctgaacatgcagactgccctcctcactaaccacagagggcagtaagttggctattgaagctttcagtccccaaaatgctctcatctcttctggatggctacataaacagaccagtgagaaccacagtaaaccctgaagggaagggaaaggaggggcagcaaagaagcagaagaaatggaaattaaagttaactaagatttttttcctagtctaatatcaatcttaacacattgatcctcatccactcgagcagctgagagccctcttaaagggcaagtgacatcgagacctgctctcggaactgtctgcaggaagactggtgttagactaggattgaagatgaagcacatcttgaagtttactgatctctgccatcggatgctgggtgaggtacagctcattcatgccttccttggctcatgcttaaaacccatcacactcctatcctcccatagttctgcacgtttctcatccactcgggcagctaagagccctcttaaagggcaagcgaccctgacacctgctttaggaactgtttgcaggagtcagtgcaggccagctccacatcctgaaggggatgccatccgggtacgaacagctcagaggctgaatggccctatcacccgggaggagcctggagggtattccatctaatcctgtggctaagcggggtggatgagggaacacacggacttgttcgagaatttgcccagcagcacgaaactacttagaagcagaaaactggggcaggacctggcgtgggagttagggagccctccactgccttctcagggatccacatgtgctcctctgtgcaggaactttcaacagcgcctcaagatagagtcacagagaacgatggcaaattccatagcactcactttttctttcctgagaaataaacagatttgggagctcagtacatcagtaatataaaagacagtgggttcagaaaaaaaaaaaaggaaaaaaatgcacaaattacaaaaaaatatgtataaagagcttcataccttttttcgtttttggttacctgtaacgttttagaattcaagaaggtttccaatgaggaaagacggaattattcagaaacagcgttcacctgatacggagaacagctccccagcgggaagtcatcatgtctcatctgacagtctagcgagctgcgtggcccctggtcactcactcactcaccctcatgggtggtctctgtgcactcatttataaaacaaacacactggaccttgccagtgattcccagatgtgactaatacccagaattccaagaactagttaaaatacagcttctgggcaccacctcctccccgttcctggtggttttggattccataattctgagcggggctcacgcatctgtattcttaaaagttcagccaggtttggggaggcttggactaggtggcctaagagaaccctttgaggcccaagcttcactacagaaatttctgtgttacccacgtgccagctactctcagggggacagtcagcaaggacccatgaggaatcataacacggggcaaagacctgtgaagatacaaggggttgctcactgcctgggcccagggttagttattcaagcaagatatgtaaagttacagatagtatttaattggttactgtgatatcatagaaataccaagaatcataaaagtaaaaaaagctgctaagttgtacataatgtttccggaatactaagaagttgctgctggtctacagagccctgggaggtgacggtgaggatggtcccaagaggcgcagctagggtcactggccccggtcctggtgcctcttgcctttgcctttcttcttcttgtcctctggccgtggctccagggcgcagacacaggcggacccgccagcgatggccttgggcaggtcgacgcccctgctccacttgtcggcctcgcggtcgtacacctgcacggtcttggagaaggcagtgttctcccagctgtagccgcccaggatgtagatgcggccctcccacactgccacgcccgactcgctgttggcgtgcagcagcggcgccacgcgggtccactggttgcactgcgggctgtaggcctccacgcccagcacgtcgaagcgctccatggactcgatgttgtcatcgctgcccccgatggagtagatgctgtcacccaggctgcacatgctgtgccagccgcgcgccgtggtcatgggccgccgctcctcccacacgtctgtccggtggtcgtagcatagcaggttcttgcggtaggggccaatttggtagtcgtggccccccgagatgtacacgaagtctttgtagatggtgcccgcgtggccgtacgtgaaccttggcaagccggccacataggaccaggagtcagtcttgggactgtacgtctctactgaagagagcgctccgttctcattccggccgccgatggccaccagcatgtcttcgatggaggcaaggtagaaatccacacggcgctggttcatggaggccacctataaagaagattggaggccgcatcccctccgttgtcccgtgagaagctgccgccggcgatgaagatgaagccccccagcaccgcgacacagtggtggctccgccgggcgggcagcggcgtctctttgacccactgctcgctcttggcgtccaggtagcaggtgtcgtcactgagctccagacaccgctcggagacctcgccgcccacaaacagcaggcgctcctggttggtgcgcagcgccgtgcgcttggtctgcatgacgggctgggccgccaggttgttgtggtagcgcacggcctcctcgatgaagccctcgcagttggcctccttgggcagcagcgagcacacggccggcttgacgcggtgcagcaggtcgttcttggggatgagcgggaagtggatgttctccagcacctggcgggcgtgggcctcgcgctcgggctgctgcgtcagccactgcagggcggcctgcaggaggtcgtgctcacactcccgctgcacctcgctgctgctcaggtagacacacagcttctgcatggagacgttctgcaggaagtcgggcgtaaaggacagcgtgccgaagtggttcaggatgaagccatcgatgaaggcatcaagccgcttgaggctgtagatggaggccagctcctgcaggtacaggtagttgtcctcgctcacctcctgctccaggtactcacagcagaagtctaccaccgtccagatctgcagcaggtgagccgtctccaggacgtagtcaatgttgccgccatccagcaccagctccccgccgtacaggaagtccaccacggccttgagcccaatgtaggaggcgccgatcagctccacctccttctggaaagcttcccgcatgccgatggtgaacatggagttgaagtagtcgctgcacacggccagcaggttgcgatgggctggcacacgctgctcatcggccaccaggacgacgtcgcagaagagcccgcggagacgctgctcgttcagccgctgcagcaccgtgcttgagtggtcggcccagcggtatacctttgatgattcgctgatcttgtatggccgagacactcgcgtctgcctgcttccctccatcattaaagagatttcagccctggcaggacgcgctacggacgcggcggggacagccccggcggcggggccgggcggtcggggcggcggggcccgggttcaggagacccccggccagcccgctgcgcagccatggctccgccaggaagtgcgag

SEQ ID NO: 9612 - RNA, 8660 nt, Homo sapiens
  source 1..8660: mol_type = other RNA
atcatacaaggacaatttcttttcttttttttttttttttttgagacagtcttactcggtcacccaggctggagtgcagtggcgcaacctcggctcactgcaacctctgcctcctgggttcaagcgattctcctgcctcagcctccggaagagctgagattacaggcgaccacgactgcctaatttttgtattttagtagagacggggtttcaccatgttggtcagggtggtctcaaactcttgacctcaggtgatccgtcccccttggcctcccagagtgctgggagtacaggcgtgagccactgcgcccggccccaaaggacaatttcttgagacccccacacaccttcagaaccacacattctgttcatgttaaaaacaagaaattaacaacctctaaagctaaggacaatgattctgtaaagtgcaagaatggttcattgtttccgcttttgtggatttcatgttaagaatactttaaaagaaagggtgggcgggagtaaaccaggaccccagtcatatatttgatcaagaaatgacccgtatggcaaaggtgagacgtggaccagccctcaggtgtctccaactctgtgcacaccactgaggtaggagctctagaagaaacgcagaccctctcaggggggttaaggtttcctcttggcaaatgagctgggggcctgagacagtcatacccacgggctgcatgcaactttgcatgcaacttcacgaaattctagagctgtatcacatcagcgatggagaagggcaagatccaagacaaagccacatgaggcgaggtcctggtgctgccatttgttgtccagcacaaatcaaggggccggaggaaagggatgaggtggaaaaccccggcaggcattctacaaaacagttattagcaaattgtatcaaaaagtatcaaaacatttcaaaaaactctaaaaactgccaggcttggcagatgcgcaggacagggtctccaagtgcccgtggcgctgccctatactccaggcatttatcctagaggccaggatgccaccccctcccctcccctcctgggcactcagaatccacggagacaccaggaggtctaaacctcatctgcagctgcccctccaggtttgggaccagtggacggggttccaaccacgggctctgacagccacaaggcccatgagatgctgctgcaccatggaggaccagggtgaaggatgaaggtcagtgactctacagggggtggtggggggtgtggcaggggtcccctcacttcccacattgctgcaagtcactgaacgatcacttggcttaggggccgaggtacactgaaccacaggtgaacacaactgagctcacaaagtaggcccctggacctcagaggatggaccccacttcccctcagcatctggatgcccacctcaaaggtgaacaccccttagggtgagtttctgggtctccatgaagtcaccttatcatgagtgagggcactcaatataaatacacacgtgtggtcctgctcagagccaggtctgaagtcccacttgatagcctcaataaaatggcagaacaataaaaataccaattgcgtgctaaccacagttgataaaataatctctgtgcatttaaaacagcaggaagtttgctataagtaacaagggttcatcagctttctactccctcccttctattattataatacatctatgtcttaagcaaacagctttccaacttgggtgaggaccaaaccccaaacttacaactaatatgaagttacaactctaattctttagaaatgagagaagtccaaacctcaatagaagcctgccatgcttattttgaaatgttaaaaaaaaaaaaagatccaggtgtcttcaaaattcaagcagaatagcttgaaacactgaaagtttaacatgatgacatgtgtggctgtttccctctcaaaatggcagcctgcaagcacctgtgccttcatcactctagtttaaaaccccacattcgtgactgtgcggttcaaatggccactgcataagcacagcccaaactctgcccatctgagttaaaaaacattttattcttttgagacagggtctcactccgtcacccaggttagagtgcagtggtgtggtcatagctcactgcagcctcaacctcccaggctcaggtgattctcccacctcagcctcctaagcagctgggactactgcatgccccaccatccctggctaatcttttgtaatttttttgtagagatggggttttgccatgttgcccaggcatggtctcttccattttcagttccattttcatgcacagtagggtgaattttcaacttaaaaagacaagtaacaaaaacctggcccgggcaccaccactgggtgcccttgtgcccatccactgaccccaacaagctcaaaaacctttcttgtcacagtgtagccaccatcaaatattagaagttgacccacaagatgaaacttgtttatcctccctttaaaagggtggtcccaaccttagtaatattagggtcaaagccatgtcaattacaaaccaccttcatagtatcaggagagacaccacaaaatatgaagcgcaggacgtcgtatgtaactcatgaggcacaagaaaatcagaatagaggccagaagctcacacatttccagggacaagtcccagaagcaaaacataaaagagctggcttaggctgaaaaccaatggctctcctctctccaaggtcaaagctatcccactccccaaatcactcacagagtctttctatgtgctctccccaacttgccccgagattcaggccaaacaactgcccgtttgttcatgacccaggctgagatggggagaacagcccacgtacaccctaccctgccttctgaggggtctacaagcaataaaacctttcccgaataggaagggggtaagctatcccaaagttggcagaagttctgcaaaacatgttttgtgggggtctgggactaggtatgagacaaacgacttttaggctcaaagaagtttggaaatgctgggttgagacttctcggaacctttcatacaccggaatgctgcagagctccaagcagagtttccagccttttggtctgtttgtttgtatgcctcgcagaacctctcaacagtttgtaagcctccagggacttcacatgcaaataactagctagctgaacatgcagactgccctcctcactaaccacagagggcagtaagttggctattgaagctttcagtccccaaaatgctctcatctcttctggatggctacataaacagaccagtgagaaccacagtaaaccctgaagggaagggaaaggaggggcagcaaagaagcagaagaaatggaaattaaagttaactaagatttttttcctagtctaatatcaatcttaacacattgatcctcatccactcgagcagctgagagccctcttaaagggcaagtgacatcgagacctgctctcggaactgtctgcaggaagactggtgttagactaggattgaagatgaagcacatcttgaagtttactgatctctgccatcggatgctgggtgaggtacagctcattcatgccttccttggctcatgcttaaaacccatcacactcctatcctcccatagttctgcacgtttctcatccactcgggcagctaagagccctcttaaagggcaagcgaccctgacacctgctttaggaactgtttgcaggagtcagtgcaggccagctccacatcctgaaggggatgccatccgggtacgaacagctcagaggctgaatggccctatcacccgggaggagcctggagggtattccatctaatcctgtggctaagcggggtggatgagggaacacacggacttgttcgagaatttgcccagcagcacgaaactacttagaagcagaaaactggggcaggacctggcgtgggagttagggagccctccactgccttctcagggatccacatgtgctcctctgtgcaggaactttcaacagcgcctcaagatagagtcacagagaacgatggcaaattccatagcactcactttttctttcctgagaaataaacagatttgggagctcagtacatcagtaatataaaagacagtgggttcagaaaaaaaaaaaaggaaaaaaatgcacaaattacaaaaaaatatgtataaagagcttcataccttttttcgtttttggttacctgtaacgttttagaattcaagaaggtttccaatgaggaaagacggaattattcagaaacagcgttcacctgatacggagaacagctccccagcgggaagtcatcatgtctcatctgacagtctagcgagctgcgtggcccctggtcactcactcactcaccctcatgggtggtctctgtgcactcatttataaaacaaacacactggaccttgccagtgattcccagatgtgactaatacccagaattccaagaactagttaaaatacagcttctgggcaccacctcctccccgttcctggtggttttggattccataattctgagcggggctcacgcatctgtattcttaaaagttcagccaggtttggggaggcttggactaggtggcctaagagaaccctttgaggcccaagcttcactacagaaatttctgtgttacccacgtgccagctactctcagggggacagtcagcaaggacccatgaggaatcataacacggggcaaagacctgtgaagatacaaggggttgctcactgcctgggcccagggttagttattcaagcaagatatgtaaagttacagatagtatttaattggttactgtgatatcatagaaataccaagaatcataaaagtaaaaaaagctgctaagttgtacataatgtttccggaatactaagaagttgctgctggtctacagagccctgggaggtgacggtgaggatggtcccaagaggcgcagctagggtcactggccccggtcctggtgcctcttgcctttgcctttcttcttcttgtcctctggccgtggctccagggcgcagacacaggcggacccgccagcgatggccttgggcaggtcgacgcccctgctccacttgtcggcctcgcggtcgtacacctgcacggtcttggagaaggcagtgttctcccagctgtagccgcccaggatgtagatgcggccctcccacactgccacgcccgactcgctgttggcgtgcagcagcggcgccacgcgggtccactggttgcactgcgggctgtaggcctccacgcccagcacgtcgaagcgctccatggactcgatgttgtcatcgctgcccccgatggagtagatgctgtcacccaggctgcacatgctgtgccagccgcgcgccgtggtcatgggccgccgctcctcccacacgtctgtccggtggtcgtagcatagcaggttcttgcggtaggggccaatttggtagtcgtggccccccgagatgtacacgaagtctttgtagatggtgcccgcgtggccgtacgtgaaccttggcaagccggccacataggaccaggagtcagtcttgggactgtacgtctctactgaagagagcgctccgttctcattccggccgccgatggccaccagcatgtcttcgatggaggcaaggtagaaatccacacggcgctggttcatggaggccacctgaataaagagggcttcttcaggtgggagctctgagcccccgaggtttcaccaagatgctctgaatccccaaaagtgggatggagacgctctgagtccccaaaagggggatggagatgctctgaacccccgaacttctctggtcatgtcgttagccgcgtggatgggaactctgtggtcacaggggtcagaattgctgatctagtggctttatgaaataaaaattcatctttcctctccccacatcagatttgtaaagttagtgctgctctgccactccgtgttaacagagcaggacgtggcattcgacaggaaattaaacagaagaggctgggcgcggtggctcacgcctgtaatcctggcactttgggaagccaaggtgggtggattacctgaggtcacggagttcgagaccagcctggccaacatggtgaaaccccgtctctactgaaaatacaaaaattagccgggcgtggtggcaggcgcctgtaattccagctactcagtaggttgaggcgccagaattgtttgaacctgggaggcagaggttgcaattagccgagatcgtgccactgcactccagcttgggtgacagaacaactctgtctcacacacacacacacaaaaagtagaagagccaacttttttttttctttttttaaacgaatccaaggcaaacacactgctgccactgctgccaggcttcgggaggaggctccaaagccagggaccctttccagtggtgacacttcgaccttggagggcagtctcagatttctgagagtaaaatcaaaaggtcagctggagtccattctgactgggttttgagctgagaacagcactgagctgggcgcgacgctgaggtgtgagtatagaggctgagatggactgtcccggggaccgagtggctggagagcgctcccagcagaaaggagacaccttccctacgccaggggcttgccagtcaacatgagctactgcactccctgtcccccacgtattcccagaaggggaatccaaaatgtggagaggacaagaatctgaaatttcctagctatgacttagccaggctgggatgagacctcaggtctgacatcaaggcccacgctcttcccagaatcaggacacaatacatgcccaagggccaggcgtgagcactagtggtctccttaaactatctcccaaaatgcttccagaggagccccacagagactccaggacctggggatgttgaaccatggatcaaacatctagacccatgctactgtccaatagggtagccacgcctcgtgcggccacatacacttacacgtcaatcggttaaagtgaaataaaattgaaaattgacttcttcagtcgcactggccacatttcaagtgctcagtcgccacatgcggctgtggctaccgtatcgggaagtacagacagacccttccatctgcacagaaagccccgccaggcagtgctgctctgaacgatgacggacccctcgaaggggtgggtcggctctccctctccctgtccaggatgtaggccccggggtattctgctcgtcactttatcatcacacctcattcagaagcaggatagttgtcaaggccccagagaggtaaggaaagtcaaggctaggttaaggaaaccgagagagtcctcaagagaaaagaaataatctggctttaatctcaccttgatccactgtttacagcgggggtcatacctataaagaagattggaggccgcatcccctccgttgtcccgtgagaagctgccgccggcgatgaagatgaagccccccagcaccgcgacacagtggtggctccgccgggcgggcagcggcgtctctttgacccactgctcgctcttggcgtccaggtagcaggtgtcgtcactgagctccagacaccgctcggagacctcgccgcccacaaacagcaggcgctcctggttggtgcgcagcgccgtgcgcttggtctgcatgacgggctgggccgccaggttgttgtggtagcgcacggcctcctcgatgaagccctcgcagttggcctccttgggcagcagcgagcacacggccggcttgacgcggtgcagcaggtcgttcttggggatgagcgggaagtggatgttctccagcacctggcgggcgtgggcctcgcgctcgggctgctgcgtcagccactgcagggcggcctgcaggaggtcgtgctcacactcccgctgcacctcgctgctgctcaggtagacacacagcttctgcatggagacgttctgcaggaagtcgggcgtaaaggacagcgtgccgaagtggttcaggatgaagccatcgatgaaggcatcaagccgcttgaggctgtagatggaggccagctcctgcaggtacaggtagttgtcctcgctcacctcctgctccaggtactcacagcagaagtctaccaccgtccagatctgcagcaggtgagccgtctccaggacgtagtcaatgttgccgccatccagcaccagctccccgccgtacaggaagtccaccacggccttgagcccaatgtaggaggcgccgatcagctccacctccttctggaaagcttcccgcatgccgatggtgaacatggagttgaagtagtcgctgcacacggccagcaggttgcgatgggctggcacacgctgctcatcggccaccaggacgacgtcgcagaagagcccgcggagacgctgctcgttcagccgctgcagcaccgtgcttgagtggtcggcccagcggtatacctttgatgattcgctgatcttgtatggccgagacactcgcgtctgcctgcttccctccatcattaaagagatttcagccctggcaggacgcgctacggacgcggcggggacagccccggcggcggggccgggcggtcggggcggcggggcccgggttcaggagacccccggccagcccgctgcgcagccatggctccgccaggaagtgcgaggccgag

SEQ ID NO: 9613 - RNA, 7188 nt, Homo sapiens
  source 1..7188: mol_type = other RNA
atcatacaaggacaatttcttttcttttttttttttttttttgagacagtcttactcggtcacccaggctggagtgcagtggcgcaacctcggctcactgcaacctctgcctcctgggttcaagcgattctcctgcctcagcctccggaagagctgagattacaggcgaccacgactgcctaatttttgtattttagtagagacggggtttcaccatgttggtcagggtggtctcaaactcttgacctcaggtgatccgtcccccttggcctcccagagtgctgggagtacaggcgtgagccactgcgcccggccccaaaggacaatttcttgagacccccacacaccttcagaaccacacattctgttcatgttaaaaacaagaaattaacaacctctaaagctaaggacaatgattctgtaaagtgcaagaatggttcattgtttccgcttttgtggatttcatgttaagaatactttaaaagaaagggtgggcgggagtaaaccaggaccccagtcatatatttgatcaagaaatgacccgtatggcaaaggtgagacgtggaccagccctcaggtgtctccaactctgtgcacaccactgaggtaggagctctagaagaaacgcagaccctctcaggggggttaaggtttcctcttggcaaatgagctgggggcctgagacagtcatacccacgggctgcatgcaactttgcatgcaacttcacgaaattctagagctgtatcacatcagcgatggagaagggcaagatccaagacaaagccacatgaggcgaggtcctggtgctgccatttgttgtccagcacaaatcaaggggccggaggaaagggatgaggtggaaaaccccggcaggcattctacaaaacagttattagcaaattgtatcaaaaagtatcaaaacatttcaaaaaactctaaaaactgccaggcttggcagatgcgcaggacagggtctccaagtgcccgtggcgctgccctatactccaggcatttatcctagaggccaggatgccaccccctcccctcccctcctgggcactcagaatccacggagacaccaggaggtctaaacctcatctgcagctgcccctccaggtttgggaccagtggacggggttccaaccacgggctctgacagccacaaggcccatgagatgctgctgcaccatggaggaccagggtgaaggatgaaggtcagtgactctacagggggtggtggggggtgtggcaggggtcccctcacttcccacattgctgcaagtcactgaacgatcacttggcttaggggccgaggtacactgaaccacaggtgaacacaactgagctcacaaagtaggcccctggacctcagaggatggaccccacttcccctcagcatctggatgcccacctcaaaggtgaacaccccttagggtgagtttctgggtctccatgaagtcaccttatcatgagtgagggcactcaatataaatacacacgtgtggtcctgctcagagccaggtctgaagtcccacttgatagcctcaataaaatggcagaacaataaaaataccaattgcgtgctaaccacagttgataaaataatctctgtgcatttaaaacagcaggaagtttgctataagtaacaagggttcatcagctttctactccctcccttctattattataatacatctatgtcttaagcaaacagctttccaacttgggtgaggaccaaaccccaaacttacaactaatatgaagttacaactctaattctttagaaatgagagaagtccaaacctcaatagaagcctgccatgcttattttgaaatgttaaaaaaaaaaaaagatccaggtgtcttcaaaattcaagcagaatagcttgaaacactgaaagtttaacatgatgacatgtgtggctgtttccctctcaaaatggcagcctgcaagcacctgtgccttcatcactctagtttaaaaccccacattcgtgactgtgcggttcaaatggccactgcataagcacagcccaaactctgcccatctgagttaaaaaacattttattcttttgagacagggtctcactccgtcacccaggttagagtgcagtggtgtggtcatagctcactgcagcctcaacctcccaggctcaggtgattctcccacctcagcctcctaagcagctgggactactgcatgccccaccatccctggctaatcttttgtaatttttttgtagagatggggttttgccatgttgcccaggcatggtctcttccattttcagttccattttcatgcacagtagggtgaattttcaacttaaaaagacaagtaacaaaaacctggcccgggcaccaccactgggtgcccttgtgcccatccactgaccccaacaagctcaaaaacctttcttgtcacagtgtagccaccatcaaatattagaagttgacccacaagatgaaacttgtttatcctccctttaaaagggtggtcccaaccttagtaatattagggtcaaagccatgtcaattacaaaccaccttcatagtatcaggagagacaccacaaaatatgaagcgcaggacgtcgtatgtaactcatgaggcacaagaaaatcagaatagaggccagaagctcacacatttccagggacaagtcccagaagcaaaacataaaagagctggcttaggctgaaaaccaatggctctcctctctccaaggtcaaagctatcccactccccaaatcactcacagagtctttctatgtgctctccccaacttgccccgagattcaggccaaacaactgcccgtttgttcatgacccaggctgagatggggagaacagcccacgtacaccctaccctgccttctgaggggtctacaagcaataaaacctttcccgaataggaagggggtaagctatcccaaagttggcagaagttctgcaaaacatgttttgtgggggtctgggactaggtatgagacaaacgacttttaggctcaaagaagtttggaaatgctgggttgagacttctcggaacctttcatacaccggaatgctgcagagctccaagcagagtttccagccttttggtctgtttgtttgtatgcctcgcagaacctctcaacagtttgtaagcctccagggacttcacatgcaaataactagctagctgaacatgcagactgccctcctcactaaccacagagggcagtaagttggctattgaagctttcagtccccaaaatgctctcatctcttctggatggctacataaacagaccagtgagaaccacagtaaaccctgaagggaagggaaaggaggggcagcaaagaagcagaagaaatggaaattaaagttaactaagatttttttcctagtctaatatcaatcttaacacattgatcctcatccactcgagcagctgagagccctcttaaagggcaagtgacatcgagacctgctctcggaactgtctgcaggaagactggtgttagactaggattgaagatgaagcacatcttgaagtttactgatctctgccatcggatgctgggtgaggtacagctcattcatgccttccttggctcatgcttaaaacccatcacactcctatcctcccatagttctgcacgtttctcatccactcgggcagctaagagccctcttaaagggcaagcgaccctgacacctgctttaggaactgtttgcaggagtcagtgcaggccagctccacatcctgaaggggatgccatccgggtacgaacagctcagaggctgaatggccctatcacccgggaggagcctggagggtattccatctaatcctgtggctaagcggggtggatgagggaacacacggacttgttcgagaatttgcccagcagcacgaaactacttagaagcagaaaactggggcaggacctggcgtgggagttagggagccctccactgccttctcagggatccacatgtgctcctctgtgcaggaactttcaacagcgcctcaagatagagtcacagagaacgatggcaaattccatagcactcactttttctttcctgagaaataaacagatttgggagctcagtacatcagtaatataaaagacagtgggttcagaaaaaaaaaaaaggaaaaaaatgcacaaattacaaaaaaatatgtataaagagcttcataccttttttcgtttttggttacctgtaacgttttagaattcaagaaggtttccaatgaggaaagacggaattattcagaaacagcgttcacctgatacggagaacagctccccagcgggaagtcatcatgtctcatctgacagtctagcgagctgcgtggcccctggtcactcactcactcaccctcatgggtggtctctgtgcactcatttataaaacaaacacactggaccttgccagtgattcccagatgtgactaatacccagaattccaagaactagttaaaatacagcttctgggcaccacctcctccccgttcctggtggttttggattccataattctgagcggggctcacgcatctgtattcttaaaagttcagccaggtttggggaggcttggactaggtggcctaagagaaccctttgaggcccaagcttcactacagaaatttctgtgttacccacgtgccagctactctcagggggacagtcagcaaggacccatgaggaatcataacacggggcaaagacctgtgaagatacaaggggttgctcactgcctgggcccagggttagttattcaagcaagatatgtaaagttacagatagtatttaattggttactgtgatatcatagaaataccaagaatcataaaagtaaaaaaagctgctaagttgtacataatgtttccggaatactaagaagttgctgctggtctacagagccctgggaggtgacggtgaggatggtcccaagaggcgcagctagggtcactggccccggtcctggtgcctcttgcctttgcctttcttcttcttgtcctctggccgtggctccagggcgcagacacaggcggacccgccagcgatggccttgggcaggtcgacgcccctgctccacttgtcggcctcgcggtcgtacacctgcacggtcttggagaaggcagtgttctcccagctgtagccgcccaggatgtagatgcggccctcccacactgccacgcccgactcgctgttggcgtgcagcagcggcgccacgcgggtccactggttgcactgcgggctgtaggcctccacgcccagcacgtcgaagcgctccatggactcgatgttgtcatcgctgcccccgatggagtagatgctgtcacccaggctgcacatgctgtgccagccgcgcgccgtggtcatgggccgccgctcctcccacacgtctgtccggtggtcgtagcatagcaggttcttgcggtaggggccaatttggtagtcgtggccccccgagatgtacacgaagtctttgtagatggtgcccgcgtggccgtacgtgaaccttggcaagccggccacataggaccaggagtcagtcttgggactgtacgtctctactgaagagagcgctccgttctcattccggccgccgatggccaccagcatgtcttcgatggaggcaaggtagaaatccacacggcgctggttcatggaggccaccttgatccactgtttacagcgggggtcatacctataaagaagattggaggccgcatcccctccgttgtcccgtgagaagctgccgccggcgatgaagatgaagccccccagcaccgcgacacagtggtggctccgccgggcgggcagcggcgtctctttgacccactgctcgctcttggcgtccaggtagcaggtgtcgtcactgagctccagacaccgctcggagacctcgccgcccacaaacagcaggcgctcctggttggtgcgcagcgccgtgcgcttggtctgcatgacgggctgggccgccaggttgttgtggtagcgcacggcctcctcgatgaagccctcgcagttggcctccttgggcagcagcgagcacacggccggcttgacgcggtgcagcaggtcgttcttggggatgagcgggaagtggatgttctccagcacctggcgggcgtgggcctcgcgctcgggctgctgcgtcagccactgcagggcggcctgcaggaggtcgtgctcacactcccgctgcacctcgctgctgctcaggtagacacacagcttctgcatggagacgttctgcaggaagtcgggcgtaaaggacagcgtgccgaagtggttcaggatgaagccatcgatgaaggcatcaagccgcttgaggctgtagatggaggccagctcctgcaggtacaggtagttgtcctcgctcacctcctgctccaggtactcacagcagaagtctaccaccgtccagatctgcagcaggtgagccgtctccaggacgtagtcaatgttgccgccatccagcaccagctccccgccgtacaggaagtccaccacggccttgagcccaatgtaggaggcgccgatcagctccacctccttctggaaagcttcccgcatgccgatggtgaacatggagttgaagtagtcgctgcacacggccagcaggttgcgatgggctggcacacgctgctcatcggccaccaggacgacgtcgcagaagagcccgcggagacgctgctcgttcagccgctgcagcaccgtgcttgagtggtcggcccagcggtatacctttgatgattcgctgatcttgtatggccgagacactcgcgtctgcctgcttccctccatcattaaagagatttcagccctagagagagttcgcggggccggaggctccctgctgtctcctgcaagtgcgtgggggtggggtctgatttccacccgtgttggacgtcagcggcctccgacgctttttggaagcaggtgaagggtcaaggccacccccaagcacagtgacaatcccaggtcactggaaaaggtcttccagtaaacatgggaccgcaggccccgtccggccgggggtttcccagagcgcctcctccccaagctccctcccgacctcagcgttggagaaagcgacgctgctgacaccggctcgccggcggggtctccggggacgccgctgtcgttcgctcggaccccgcagcccaggcggaactc

SEQ ID NO: 9614 - RNA, 6974 nt, Homo sapiens
  source 1..6974: mol_type = other RNA
atcatacaaggacaatttcttttcttttttttttttttttttgagacagtcttactcggtcacccaggctggagtgcagtggcgcaacctcggctcactgcaacctctgcctcctgggttcaagcgattctcctgcctcagcctccggaagagctgagattacaggcgaccacgactgcctaatttttgtattttagtagagacggggtttcaccatgttggtcagggtggtctcaaactcttgacctcaggtgatccgtcccccttggcctcccagagtgctgggagtacaggcgtgagccactgcgcccggccccaaaggacaatttcttgagacccccacacaccttcagaaccacacattctgttcatgttaaaaacaagaaattaacaacctctaaagctaaggacaatgattctgtaaagtgcaagaatggttcattgtttccgcttttgtggatttcatgttaagaatactttaaaagaaagggtgggcgggagtaaaccaggaccccagtcatatatttgatcaagaaatgacccgtatggcaaaggtgagacgtggaccagccctcaggtgtctccaactctgtgcacaccactgaggtaggagctctagaagaaacgcagaccctctcaggggggttaaggtttcctcttggcaaatgagctgggggcctgagacagtcatacccacgggctgcatgcaactttgcatgcaacttcacgaaattctagagctgtatcacatcagcgatggagaagggcaagatccaagacaaagccacatgaggcgaggtcctggtgctgccatttgttgtccagcacaaatcaaggggccggaggaaagggatgaggtggaaaaccccggcaggcattctacaaaacagttattagcaaattgtatcaaaaagtatcaaaacatttcaaaaaactctaaaaactgccaggcttggcagatgcgcaggacagggtctccaagtgcccgtggcgctgccctatactccaggcatttatcctagaggccaggatgccaccccctcccctcccctcctgggcactcagaatccacggagacaccaggaggtctaaacctcatctgcagctgcccctccaggtttgggaccagtggacggggttccaaccacgggctctgacagccacaaggcccatgagatgctgctgcaccatggaggaccagggtgaaggatgaaggtcagtgactctacagggggtggtggggggtgtggcaggggtcccctcacttcccacattgctgcaagtcactgaacgatcacttggcttaggggccgaggtacactgaaccacaggtgaacacaactgagctcacaaagtaggcccctggacctcagaggatggaccccacttcccctcagcatctggatgcccacctcaaaggtgaacaccccttagggtgagtttctgggtctccatgaagtcaccttatcatgagtgagggcactcaatataaatacacacgtgtggtcctgctcagagccaggtctgaagtcccacttgatagcctcaataaaatggcagaacaataaaaataccaattgcgtgctaaccacagttgataaaataatctctgtgcatttaaaacagcaggaagtttgctataagtaacaagggttcatcagctttctactccctcccttctattattataatacatctatgtcttaagcaaacagctttccaacttgggtgaggaccaaaccccaaacttacaactaatatgaagttacaactctaattctttagaaatgagagaagtccaaacctcaatagaagcctgccatgcttattttgaaatgttaaaaaaaaaaaaagatccaggtgtcttcaaaattcaagcagaatagcttgaaacactgaaagtttaacatgatgacatgtgtggctgtttccctctcaaaatggcagcctgcaagcacctgtgccttcatcactctagtttaaaaccccacattcgtgactgtgcggttcaaatggccactgcataagcacagcccaaactctgcccatctgagttaaaaaacattttattcttttgagacagggtctcactccgtcacccaggttagagtgcagtggtgtggtcatagctcactgcagcctcaacctcccaggctcaggtgattctcccacctcagcctcctaagcagctgggactactgcatgccccaccatccctggctaatcttttgtaatttttttgtagagatggggttttgccatgttgcccaggcatggtctcttccattttcagttccattttcatgcacagtagggtgaattttcaacttaaaaagacaagtaacaaaaacctggcccgggcaccaccactgggtgcccttgtgcccatccactgaccccaacaagctcaaaaacctttcttgtcacagtgtagccaccatcaaatattagaagttgacccacaagatgaaacttgtttatcctccctttaaaagggtggtcccaaccttagtaatattagggtcaaagccatgtcaattacaaaccaccttcatagtatcaggagagacaccacaaaatatgaagcgcaggacgtcgtatgtaactcatgaggcacaagaaaatcagaatagaggccagaagctcacacatttccagggacaagtcccagaagcaaaacataaaagagctggcttaggctgaaaaccaatggctctcctctctccaaggtcaaagctatcccactccccaaatcactcacagagtctttctatgtgctctccccaacttgccccgagattcaggccaaacaactgcccgtttgttcatgacccaggctgagatggggagaacagcccacgtacaccctaccctgccttctgaggggtctacaagcaataaaacctttcccgaataggaagggggtaagctatcccaaagttggcagaagttctgcaaaacatgttttgtgggggtctgggactaggtatgagacaaacgacttttaggctcaaagaagtttggaaatgctgggttgagacttctcggaacctttcatacaccggaatgctgcagagctccaagcagagtttccagccttttggtctgtttgtttgtatgcctcgcagaacctctcaacagtttgtaagcctccagggacttcacatgcaaataactagctagctgaacatgcagactgccctcctcactaaccacagagggcagtaagttggctattgaagctttcagtccccaaaatgctctcatctcttctggatggctacataaacagaccagtgagaaccacagtaaaccctgaagggaagggaaaggaggggcagcaaagaagcagaagaaatggaaattaaagttaactaagatttttttcctagtctaatatcaatcttaacacattgatcctcatccactcgagcagctgagagccctcttaaagggcaagtgacatcgagacctgctctcggaactgtctgcaggaagactggtgttagactaggattgaagatgaagcacatcttgaagtttactgatctctgccatcggatgctgggtgaggtacagctcattcatgccttccttggctcatgcttaaaacccatcacactcctatcctcccatagttctgcacgtttctcatccactcgggcagctaagagccctcttaaagggcaagcgaccctgacacctgctttaggaactgtttgcaggagtcagtgcaggccagctccacatcctgaaggggatgccatccgggtacgaacagctcagaggctgaatggccctatcacccgggaggagcctggagggtattccatctaatcctgtggctaagcggggtggatgagggaacacacggacttgttcgagaatttgcccagcagcacgaaactacttagaagcagaaaactggggcaggacctggcgtgggagttagggagccctccactgccttctcagggatccacatgtgctcctctgtgcaggaactttcaacagcgcctcaagatagagtcacagagaacgatggcaaattccatagcactcactttttctttcctgagaaataaacagatttgggagctcagtacatcagtaatataaaagacagtgggttcagaaaaaaaaaaaaggaaaaaaatgcacaaattacaaaaaaatatgtataaagagcttcataccttttttcgtttttggttacctgtaacgttttagaattcaagaaggtttccaatgaggaaagacggaattattcagaaacagcgttcacctgatacggagaacagctccccagcgggaagtcatcatgtctcatctgacagtctagcgagctgcgtggcccctggtcactcactcactcaccctcatgggtggtctctgtgcactcatttataaaacaaacacactggaccttgccagtgattcccagatgtgactaatacccagaattccaagaactagttaaaatacagcttctgggcaccacctcctccccgttcctggtggttttggattccataattctgagcggggctcacgcatctgtattcttaaaagttcagccaggtttggggaggcttggactaggtggcctaagagaaccctttgaggcccaagcttcactacagaaatttctgtgttacccacgtgccagctactctcagggggacagtcagcaaggacccatgaggaatcataacacggggcaaagacctgtgaagatacaaggggttgctcactgcctgggcccagggttagttattcaagcaagatatgtaaagttacagatagtatttaattggttactgtgatatcatagaaataccaagaatcataaaagtaaaaaaagctgctaagttgtacataatgtttccggaatactaagaagttgctgctggtctacagagccctgggaggtgacggtgaggatggtcccaagaggcgcagctagggtcactggccccggtcctggtgcctcttgcctttgcctttcttcttcttgtcctctggccgtggctccagggcgcagacacaggcggacccgccagcgatggccttgggcaggtcgacgcccctgctccacttgtcggcctcgcggtcgtacacctgcacggtcttggagaaggcagtgttctcccagctgtagccgcccaggatgtagatgcggccctcccacactgccacgcccgactcgctgttggcgtgcagcagcggcgccacgcgggtccactggttgcactgcgggctgtaggcctccacgcccagcacgtcgaagcgctccatggactcgatgttgtcatcgctgcccccgatggagtagatgctgtcacccaggctgcacatgctgtgccagccgcgcgccgtggtcatgggccgccgctcctcccacacgtctgtccggtggtcgtagcatagcaggttcttgcggtaggggccaatttggtagtcgtggccccccgagatgtacacgaagtctttgtagatggtgcccgcgtggccgtacgtgaaccttggcaagccggccacataggaccaggagtcagtcttgggactgtacgtctctactgaagagagcgctccgttctcattccggccgccgatggccaccagcatgtcttcgatggaggcaaggtagaaatccacacggcgctggttcatggaggccaccttgatccactgtttacagcgggggtcatacctataaagaagattggaggccgcatcccctccgttgtcccgtgagaagctgccgccggcgatgaagatgaagccccccagcaccgcgacacagtggtggctccgccgggcgggcagcggcgtctctttgacccactgctcgctcttggcgtccaggtagcaggtgtcgtcactgagctccagacaccgctcggagacctcgccgcccacaaacagcaggcgctcctggttggtgcgcagcgccgtgcgcttggtctgcatgacgggctgggccgccaggttgttgtggtagcgcacggcctcctcgatgaagccctcgcagttggcctccttgggcagcagcgagcacacggccggcttgacgcggtgcagcaggtcgttcttggggatgagcgggaagtggatgttctccagcacctggcgggcgtgggcctcgcgctcgggctgctgcgtcagccactgcagggcggcctgcaggaggtcgtgctcacactcccgctgcacctcgctgctgctcaggtagacacacagcttctgcatggagacgttctgcaggaagtcgggcgtaaaggacagcgtgccgaagtggttcaggatgaagccatcgatgaaggcatcaagccgcttgaggctgtagatggaggccagctcctgcaggtacaggtagttgtcctcgctcacctcctgctccaggtactcacagcagaagtctaccaccgtccagatctgcagcaggtgagccgtctccaggacgtagtcaatgttgccgccatccagcaccagctccccgccgtacaggaagtccaccacggccttgagcccaatgtaggaggcgccgatcagctccacctccttctggaaagcttcccgcatgccgatggtgaacatggagttgaagtagtcgctgcacacggccagcaggttgcgatgggctggcacacgctgctcatcggccaccaggacgacgtcgcagaagagcccgcggagacgctgctcgttcagccgctgcagcaccgtgcttgagtggtcggcccagcggtatacctttgatgattcgctgatcttgtatggccgagacactcgcgtctgcctgcttccctccatcattaaagagatttcagccctggcaggacgcgctacggacgcggcggggacagccccggcggcggggccgggcggtcggggcggcggggcccgggttcaggagacccccggccagcccgctgcgcagccatggctccgccaggaagtgcgaggccgag

SEQ ID NO: 9615 - RNA, 4630 nt, Homo sapiens
  source 1..4630: mol_type = other RNA
atcatgatgggctcctcggtgtcggcgctgcctgggccctcagtggcctccacgccgtcgcagctgtcgccctccgagctgggcgccgcccggccgctgcgggccgagggtgagtcgctggcgcccgcctggccctgactcccggcctgaatttcctcaatgaacagttctctgcggatccgagacctgtagttgtggaaccagttgatgacggtgctggttttcaggttgagctgggtggcgaggtcttcgatggtttttggtgacgggtatggcttttgctgatacgctcgtttcagcgcctccttctcctccggagccagcaccacccggggtttcttcagctggtgctggggctgggggctggcgccctggctgtactcggtgccgacagagggcggttcgcagggctggctgtcactgactgagctgtgccgccgcttcatgtaggctttcttctccatccgtttcatgtccatcagcttctccacattgttggggtcgttcagccacagctgcatccggacgaagggctctcgtcctttcagactgagcttatgccagggtttggggcgggcaaggaggtcagagacagagccttgggtgagccctaagatggtctccccaaataagcgctggccgaggttgttgtccgtcagcacctccttcacccgcttggttatgccgtaggtgtccagctccggggacatggctactaattcttggatgctgagggccgagtgtccggagagaggcagcggggttgtgggctgggagtcggatgctggcgggtcactgggctctggtggcttgctgtccttgctcgcctcgatggggggacagggctgctggaccagctcggtcaggctcttcaccgactcactggaactcatcggggactcaggggcagggctgcagctggcggaggtctttggagtgctttctgagctcacacagccctgctgcagcgggtcctggagcgatgtcacggagtggaggactggcccttgctgctggccctggacgggtagaacaccctggcctagctcgccgttcagccagagctgcatccggatgaagggttctcggcctttctgcgtcagcttgctccatggcttcggtcgggacagcatgtcgctgacgctgccctgggacaggcccagcaccttctccccgaagattctctggcagatgccgttcttggccagcttttccttaacctgccgggtgagctcgatggtgtccacctcctggtacatgtagacctcgtactgctcgggggtcagcggggggaccgagggcttggtgggcttggacatgggcacgatcggggaggatggcagggggctgttctgtggtgtctcgctgcggctggccccggtcagactcagctctgagctctgggagtatggggactcagcgctgggccactccttccagtactctgacgacgagggtccctggagctgactgcgctcggcccgaggctggctgccacctccgctgccaccgctgcccttctctttcccgccgcccgtttcttcggccttggcctcctcggaggaggcggcatttcttctctccggctgcaccgcgctccaccagtggtccttccaggcaccgctgcggcccacctcatttttcacctgtctcaggaccccttgtgcacaatcggctgctccctgggggtccagcccgggggcgtcctgggcctcctttttgagggccggggggttcggcagagcagaggcaccggcctcaggagctgcggagggcttcttcagggagatggcgagaggtgggtagctggacacggtgggcatgggcgaggtggacagaagcttgggggtgaggatggtgatgtcactctgggacagtggtgcctgctttaaggcagggtcgagggcagcctgctgggcctccatctcccggcgggcttgctgcaggatggagcggatggcgtcatcagagttcccgctgccggatgcggaggaaggctgggccggctcagttttctgcacttggagctccctcttggcttgctctaggatggacttgatggcttcatcagagccagtctccgaggctcggatccgggtggtgatgttaccttcagacccatttcttcgtttcggtacttcctgaaatagtctgttcaggctctggcctggattctctctttgtctgccttggatgctacggagggccaggatgttctgctcatcggagaggaactgtttcatcttgtgaaatggctccttgccacgaacagtcagtttattccatggcttgggccgggccagaatctcgctcacggacccttgagacagtcccaacacataatgtccgaaaatacgttgtccgatattgtgcttaatcagctgctctttgacctgccgggcgatttctgcagtgtccatctcctcgccctcggagacgctcccagcactttctgactggctgggggatggggccatgccattgacatctgggctttgttgtaatggactttgggaagatatggagtttgtgctgtatggacctgttgaaaaaatcatgcttgtgcttccggcttcctgcatagccttggagtagaaggactgcattagctgccgctggagaagagagtttagtgcaaattttcctgtagaagccaggggtaggctggggcttgccagggatgagctgaaaaagtcttgacttaaccccgctggtgagaactggtgtgtaccattagtattggaagcctgctcccccgggttgcggggcaactgagaaggagggggggccggcaaagatcccgggcgccgactttcaggctggtctttccctttcctcctggctgacccgctcaggtcgctgttggagatgcgcagcgcggcgttctcggactgcagcgagcggttcttctccagcaacagcacctccaggggcttggccgcatcctgtgtcccagcgccctcggacggtgcaaactccatggacttcagaatgttcagctctttcttcacctcttcatagtcagcctggcctttgagtttttcttccagttgtttgagtgtgctgtttttggcgctcagctgctgctcaagctgtgagatctggctggccgaattctcccgcagcttggtgaggctggcctggagtctctgcacgtcctccaccagctgtgcgatctcccgctccttggcggccaactcaacttctaggctggagcgggtcagcacctctatggcctgctccacgtctggtgccttctggatctgtgaggccagctggagggagtgattggccgatgagagctgttcccttaaggtctccgcctctctctgagccacctctgccctctggtttgccctttcaaggtccgtcatgatcatttcaatctcgtcggcctttgcagtagtttcttcatcgtatttggttttcaggtcaaataattctgttcgagttttttccagggctgtttgtaggctctgaaccttatgctcagcttcctccagctttgaggtggtggacatctgtgtctcctgcagctttctctccttttctgcaaagtcattctgtaacttctgttccttctcaagagctatggtttcggcttggttcttcagtgtctgttcatattctcggattttctctttaagtgcttttatcgtaacctcttgatttttcacttcagcaaattccttgttgtattcttccagagtttccctaagtttctggttctctgtttcaatatcgtgcaggcgctgcactttgagctggagttgctgtccgagatccaaagctggtacgggatctgggacgtcaatcaatcttttgtagacattcaagaaagctgcttcagcttccttgcttcttttactcagtgcatcaatctctccttggaaactcttcagcagcggcgctacctgcttgcgcaaatcctctggagtgttcttcttgaactcccggctctgttcgataagccgctttctggactgctcactttcatcctgccggttcgccaataccgttgcggtggcatcgagttctctcttcaacctggctccggctacgcacaacatccacctggcagagtcccggggctgtcccggcgccgcgggcgccgagctggcacgtgcggggcggaccctaagggtgcgccgctcctccgggcggggggtggcaggcaggcactcgccccttgggcacggcggcgactcgggcgcgggccggggagccccggcacggtccccccgcggcgccggggactccgcgcgcggaccaccgcccggcatgccacggtcccaacgggcccccggggctctgctttcgagaacccggcccgagaaggcatctccgagcgcacccgccgcgcgctccatggcgggccctgcagagagggcagaagccccgaggggacgcaaggaagggacccggcgccgcaggtcaccgggggccgccggagcccccaggcgcgcggcgatcgcggctcggaccggcggcggggaggcagcgtacactgcccgggcacccgggggaacagcttggggcctgcctaggggaaagttgcagcctcctcctcccgcgcccgcacccggcggtccgggacaccgggacccagcgacactgcgcgcggggcacc

SEQ ID NO: 9616 - RNA, 4074 nt, Homo sapiens
  source 1..4074: mol_type = other RNA
atcatgatgggctcctcggtgtcggcgctgcctgggccctcagtggcctccacgccgtcgcagctgtcgccctccgagctgggcgccgcccggccgctgcgggccgagggtgagtcgctggcgcccgcctggccctgactcccggcctgaatttcctcaatgaacagttctctgcggatccgagacctgtagttgtggaaccagttgatgacggtgctggttttcaggttgagctgggtggcgaggtcttcgatggtttttggtgacgggtatggcttttgctgatacgctcgtttcagcgcctccttctcctccggagccagcaccacccggggtttcttcagctggtgctggggctgggggctggcgccctggctgtactcggtgccgacagagggcggttcgcagggctggctgtcactgactgagctgtgccgccgcttcatgtaggctttcttctccatccgtttcatgtccatcagcttctccacattgttggggtcgttcagccacagctgcatccggacgaagggctctcgtcctttcagactgagcttatgccagggtttggggcgggcaaggaggtcagagacagagccttgggtgagccctaagatggtctccccaaataagcgctggccgaggttgttgtccgtcagcacctccttcacccgcttggttatgccgtaggtgtccagctccggggacatggctactaattcttggatgctgagggccgagtgtccggagagaggcagcggggttgtgggctgggagtcggatgctggcgggtcactgggctctggtggcttgctgtccttgctcgcctcgatggggggacagggctgctggaccagctcggtcaggctcttcaccgactcactggaactcatcggggactcaggggcagggctgcagctggcggaggtctttggagtgctttctgagctcacacagccctgctgcagcgggtcctggagcgatgtcacggagtggaggactggcccttgctgctggccctggacgggtagaacaccctggcctagctcgccgttcagccagagctgcatccggatgaagggttctcggcctttctgcgtcagcttgctccatggcttcggtcgggacagcatgtcgctgacgctgccctgggacaggcccagcaccttctccccgaagattctctggcagatgccgttcttggccagcttttccttaacctgccgggtgagctcgatggtgtccacctcctggtacatgtagacctcgtactgctcgggggtcagcggggggaccgagggcttggtgggcttggacatgggcacgatcggggaggatggcagggggctgttctgtggtgtctcgctgcggctggccccggtcagactcagctctgagctctgggagtatggggactcagcgctgggccactccttccagtactctgacgacgagggtccctggagctgactgcgctcggcccgaggctggctgccacctccgctgccaccgctgcccttctctttcccgccgcccgtttcttcggccttggcctcctcggaggaggcggcatttcttctctccggctgcaccgcgctccaccagtggtccttccaggcaccgctgcggcccacctcatttttcacctgtctcaggaccccttgtgcacaatcggctgctccctgggggtccagcccgggggcgtcctgggcctcctttttgagggccggggggttcggcagagcagaggcaccggcctcaggagctgcggagggcttcttcagggagatggcgagaggtgggtagctggacacggtgggcatgggcgaggtggacagaagcttgggggtgaggatggtgatgtcactctgggacagtggtgcctgctttaaggcagggtcgagggcagcctgctgggcctccatctcccggcgggcttgctgcaggatggagcggatggcgtcatcagagttcccgctgccggatgcggaggaaggctgggccggctctgcagttttctgcacttggagctccctcttggcttgctctaggatggacttgatggcttcatcagagccagtctccgaggctcggatccgggtggtgatgttacctctttgtctgccttggatgctacggagggccaggatgttctgctcatcggagaggaactgtttcatcttgtgaaatggctccttgccacgaacagtcagtttattccatggcttgggccgggccagaatctcgctcacggacccttgagacagtcccaacacataatgtccgaaaatacgttgtccgatattgtgcttaatcagctgctctttgacctgccgggcgatttctgcagtgtccatctcctcgccctcggagacgctcccagcactttctgactggctgggggatggggccatgccattgacatctgggctttgttgtaatggactttgggaagatatggagtttgtgctgtatggacctgttgaaaaaatcatgcttgtgcttccggcttcctgcatagccttggagtagaaggactgcattagctgccgctggagaagagagtttagtgcaaattttcctgtagaagccaggggtaggctggggcttgccagggatgagctgaaaaagtcttgacttaaccccgctggtgagaactggtgtgtaccattagtattggaagcctgctcccccgggttgcggggcaactgagaaggagggggggccggcaaagatcccgggcgccgactttcaggctggtctttccctttcctcctggctgacccgctcaggtcgctgttggagatgcgcagcgcggcgttctcggactgcagcgagcggttcttctccagcaacagcacctccaggggcttggccgcatcctgtgtcccagcgccctcggacggtgcaaactccatggacttcagaatgttcagctctttcttcacctcttcatagtcagcctggcctttgagtttttcttccagttgtttgagtgtgctgtttttggcgctcagctgctgctcaagctgtgagatctggctggccgaattctcccgcagcttggtgaggctggcctggagtctctgcacgtcctccaccagctgtgcgatctcccgctccttggcggccaactcaacttctaggctggagcgggtcagcacctctatggccacgtctggtgccttctggatctgtgaggccagctggagggagtgattggccgatgagagctgttcccttaaggtctccgcctctctctgagccacctctgccctctggtttgccctttcaaggtccgtcatgatcatttcaatctcgtcggcctttgcagtagtttcttcatcgtatttggttttcaggtcaaataattctgttcgagttttttccagggctgtttgtaggctctgaaccttatgctcagcttcctccagctttgaggtggtggacatctgtgtctcctgcagctttctctccttttctgcaaagtcattctgtaacttctgttccttctcaagagctatggtttcggcttggttcttcagtgtctgttcatattctcggattttctctttaagtgcttttatcgtaacctcttgatttttcacttcagcaaattccttgttgtattcttccagagtttccctaagtttctggttctctgtttcaatatcgtgcaggcgctgcactttgagctggagttgctgtccgagatccaaagctggtacgggatctgggacgtcaatcaatcttttgtagacattcaagaaagctgcttcagcttccttgcttcttttactcagtgcatcaatctctccttggaaactcttcagcagcggcgctacctgcttgcgcaaatcctctggagtgttcttcttgaactcccggctctgttcgataagccgctttctggactgctcactttcatcctgccggttcgccaataccgttgcggtggcatcgagttctctctgcagctgctgtaaatcaaagcgcttccaatattgaaacatcgatcccacattggccgccatcttgagacatattgagacggagtgagcggctgatagagag

SEQ ID NO: 9617 - RNA, 4566 nt, Homo sapiens
  source 1..4566: mol_type = other RNA
atcatgatgggctcctcggtgtcggcgctgcctgggccctcagtggcctccacgccgtcgcagctgtcgccctccgagctgggcgccgcccggccgctgcgggccgagggtgagtcgctggcgcccgcctggccctgactcccggcctgaatttcctcaatgaacagttctctgcggatccgagacctgtagttgtggaaccagttgatgacggtgctggttttcaggttgagctgggtggcgaggtcttcgatggtttttggtgacgggtatggcttttgctgatacgctcgtttcagcgcctccttctcctccggagccagcaccacccggggtttcttcagctggtgctggggctgggggctggcgccctggctgtactcggtgccgacagagggcggttcgcagggctggctgtcactgactgagctgtgccgccgcttcatgtaggctttcttctccatccgtttcatgtccatcagcttctccacattgttggggtcgttcagccacagctgcatccggacgaagggctctcgtcctttcagactgagcttatgccagggtttggggcgggcaaggaggtcagagacagagccttgggtgagccctaagatggtctccccaaataagcgctggccgaggttgttgtccgtcagcacctccttcacccgcttggttatgccgtaggtgtccagctccggggacatggctactaattcttggatgctgagggccgagtgtccggagagaggcagcggggttgtgggctgggagtcggatgctggcgggtcactgggctctggtggcttgctgtccttgctcgcctcgatggggggacagggctgctggaccagctcggtcaggctcttcaccgactcactggaactcatcggggactcaggggcagggctgcagctggcggaggtctttggagtgctttctgagctcacacagccctgctgcagcgggtcctggagcgatgtcacggagtggaggactggcccttgctgctggccctggacgggtagaacaccctggcctagctcgccgttcagccagagctgcatccggatgaagggttctcggcctttctgcgtcagcttgctccatggcttcggtcgggacagcatgtcgctgacgctgccctgggacaggcccagcaccttctccccgaagattctctggcagatgccgttcttggccagcttttccttaacctgccgggtgagctcgatggtgtccacctcctggtacatgtagacctcgtactgctcgggggtcagcggggggaccgagggcttggtgggcttggacatgggcacgatcggggaggatggcagggggctgttctgtggtgtctcgctgcggctggccccggtcagactcagctctgagctctgggagtatggggactcagcgctgggccactccttccagtactctgacgacgagggtccctggagctgactgcgctcggcccgaggctggctgccacctccgctgccaccgctgcccttctctttcccgccgcccgtttcttcggccttggcctcctcggaggaggcggcatttcttctctccggctgcaccgcgctccaccagtggtccttccaggcaccgctgcggcccacctcatttttcacctgtctcaggaccccttgtgcacaatcggctgctccctgggggtccagcccgggggcgtcctgggcctcctttttgagggccggggggttcggcagagcagaggcaccggcctcaggagctgcggagggcttcttcagggagatggcgagaggtgggtagctggacacggtgggcatgggcgaggtggacagaagcttgggggtgaggatggtgatgtcactctgggacagtggtgcctgctttaaggcagggtcgagggcagcctgctgggcctccatctcccggcgggcttgctgcaggatggagcggatggcgtcatcagagttcccgctgccggatgcggaggaaggctgggccggctctgcagttttctgcacttggagctccctcttggcttgctctaggatggacttgatggcttcatcagagccagtctccgaggctcggatccgggtggtgatgttacctctttgtctgccttggatgctacggagggccaggatgttctgctcatcggagaggaactgtttcatcttgtgaaatggctccttgccacgaacagtcagtttattccatggcttgggccgggccagaatctcgctcacggacccttgagacagtcccaacacataatgtccgaaaatacgttgtccgatattgtgcttaatcagctgctctttgacctgccgggcgatttctgcagtgtccatctcctcgccctcggagacgctcccagcactttctgactggctgggggatggggccatgccattgacatctgggctttgttgtaatggactttgggaagatatggagtttgtgctgtatggacctgttgaaaaaatcatgcttgtgcttccggcttcctgcatagccttggagtagaaggactgcattagctgccgctggagaagagagtttagtgcaaattttcctgtagaagccaggggtaggctggggcttgccagggatgagctgaaaaagtcttgacttaaccccgctggtgagaactggtgtgtaccattagtattggaagcctgctcccccgggttgcggggcaactgagaaggagggggggccggcaaagatcccgggcgccgactttcaggctggtctttccctttcctcctggctgacccgctcaggtcgctgttggagatgcgcagcgcggcgttctcggactgcagcgagcggttcttctccagcaacagcacctccaggggcttggccgcatcctgtgtcccagcgccctcggacggtgcaaactccatggacttcagaatgttcagctctttcttcacctcttcatagtcagcctggcctttgagtttttcttccagttgtttgagtgtgctgtttttggcgctcagctgctgctcaagctgtgagatctggctggccgaattctcccgcagcttggtgaggctggcctggagtctctgcacgtcctccaccagctgtgcgatctcccgctccttggcggccaactcaacttctaggctggagcgggtcagcacctctatggcctgctccacgtctggtgccttctggatctgtgaggccagctggagggagtgattggccgatgagagctgttcccttaaggtctccgcctctctctgagccacctctgccctctggtttgccctttcaaggtccgtcatgatcatttcaatctcgtcggcctttgcagtagtttcttcatcgtatttggttttcaggtcaaataattctgttcgagttttttccagggctgtttgtaggctctgaaccttatgctcagcttcctccagctttgaggtggtggacatctgtgtctcctgcagctttctctccttttctgcaaagtcattctgtaacttctgttccttctcaagagctatggtttcggcttggttcttcagtgtctgttcatattctcggattttctctttaagtgcttttatcgtaacctcttgatttttcacttcagcaaattccttgttgtattcttccagagtttccctaagtttctggttctctgtttcaatatcgtgcaggcgctgcactttgagctggagttgctgtccgagatccaaagctggtacgggatctgggacgtcaatcaatcttttgtagacattcaagaaagctgcttcagcttccttgcttcttttactcagtgcatcaatctctccttggaaactcttcagcagcggcgctacctgcttgcgcaaatcctctggagtgttcttcttgaactcccggctctgttcgataagccgctttctggactgctcactttcatcctgccggttcgccaataccgttgcggtggcatcgagttctctcttcaacctggctccggctacgcacaacatccacctggcagagtcccggggctgtcccggcgccgcgggcgccgagctggcacgtgcggggcggaccctaagggtgcgccgctcctccgggcggggggtggcaggcaggcactcgccccttgggcacggcggcgactcgggcgcgggccggggagccccggcacggtccccccgcggcgccggggactccgcgcgcggaccaccgcccggcatgccacggtcccaacgggcccccggggctctgctttcgagaacccggcccgagaaggcatctccgagcgcacccgccgcgcgctccatggcgggccctgcagagagggcagaagccccgaggggacgcaaggaagggacccggcgccgcaggtcaccgggggccgccggagcccccaggcgcgcggcgatcgcggctcggaccggcggcggggaggcagcgtacactgcccgggcacccgggggaacagcttggggcctgcctaggggaaagttgcagcctcctcctcccgcgcccgcacccggcggtccgggacaccgggacccagcgacactgcgcgcggggcac

SEQ ID NO: 9618 - RNA, 4322 nt, Homo sapiens
  source 1..4322: mol_type = other RNA
atcatgatgggctcctcggtgtcggcgctgcctgggccctcagtggcctccacgccgtcgcagctgtcgccctccgagctgggcgccgcccggccgctgcgggccgagggtgagtcgctggcgcccgcctggccctgactcccggcctgaatttcctcaatgaacagttctctgcggatccgagacctgtagttgtggaaccagttgatgacggtgctggttttcaggttgagctgggtggcgaggtcttcgatggtttttggtgacgggtatggcttttgctgatacgctcgtttcagcgcctccttctcctccggagccagcaccacccggggtttcttcagctggtgctggggctgggggctggcgccctggctgtactcggtgccgacagagggcggttcgcagggctggctgtcactgactgagctgtgccgccgcttcatgtaggctttcttctccatccgtttcatgtccatcagcttctccacattgttggggtcgttcagccacagctgcatccggacgaagggctctcgtcctttcagactgagcttatgccagggtttggggcgggcaaggaggtcagagacagagccttgggtgagccctaagatggtctccccaaataagcgctggccgaggttgttgtccgtcagcacctccttcacccgcttggttatgccgtaggtgtccagctccggggacatggctactaattcttggatgctgagggccgagtgtccggagagaggcagcggggttgtgggctgggagtcggatgctggcgggtcactgggctctggtggcttgctgtccttgctcgcctcgatggggggacagggctgctggaccagctcggtcaggctcttcaccgactcactggaactcatcggggactcaggggcagggctgcagctggcggaggtctttggagtgctttctgagctcacacagccctgctgcagcgggtcctggagcgatgtcacggagtggaggactggcccttgctgctggccctggacgggtagaacaccctggcctagctcgccgttcagccagagctgcatccggatgaagggttctcggcctttctgcgtcagcttgctccatggcttcggtcgggacagcatgtcgctgacgctgccctgggacaggcccagcaccttctccccgaagattctctggcagatgccgttcttggccagcttttccttaacctgccgggtgagctcgatggtgtccacctcctggtacatgtagacctcgtactgctcgggggtcagcggggggaccgagggcttggtgggcttggacatgggcacgatcggggaggatggcagggggctgttctgtggtgtctcgctgcggctggccccggtcagactcagctctgagctctgggagtatggggactcagcgctgggccactccttccagtactctgacgacgagggtccctggagctgactgcgctcggcccgaggctggctgccacctccgctgccaccgctgcccttctctttcccgccgcccgtttcttcggccttggcctcctcggaggaggcggcatttcttctctccggctgcaccgcgctccaccagtggtccttccaggcaccgctgcggcccacctcatttttcacctgtctcaggaccccttgtgcacaatcggctgctccctgggggtccagcccgggggcgtcctgggcctcctttttgagggccggggggttcggcagagcagaggcaccggcctcaggagctgcggagggcttcttcagggagatggcgagaggtgggtagctggacacggtgggcatgggcgaggtggacagaagcttgggggtgaggatggtgatgtcactctgggacagtggtgcctgctttaaggcagggtcgagggcagcctgctgggcctccatctcccggcgggcttgctgcaggatggagcggatggcgtcatcagagttcccgctgccggatgcggaggaaggctgggccggctctgcagttttctgcacttggagctccctcttggcttgctctaggatggacttgatggcttcatcagagccagtctccgaggctcggatccgggtggtgatgttaccttcagacccatttcttcgtttcggtacttcctgaaatagtctgttcaggctctggcctggattctctctttgtctgccttggatgctacggagggccaggatgttctgctcatcggagaggaactgtttcatcttgtgaaatggctccttgccacgaacagtcagtttattccatggcttgggccgggccagaatctcgctcacggacccttgagacagtcccaacacataatgtccgaaaatacgttgtccgatattgtgcttaatcagctgctctttgacctgccgggcgatttctgcagtgtccatctcctcgccctcggagacgctcccagcactttctgactggctgggggatggggccatgccattgacatctgggctttgttgtaatggactttgggaagatatggagtttgtgctgtatggaccgctcaggtcgctgttggagatgcgcagcgcggcgttctcggactgcagcgagcggttcttctccagcaacagcacctccaggggcttggccgcatcctgtgtcccagcgccctcggacggtgcaaactccatggacttcagaatgttcagctctttcttcacctcttcatagtcagcctggcctttgagtttttcttccagttgtttgagtgtgctgtttttggcgctcagctgctgctcaagctgtgagatctggctggccgaattctcccgcagcttggtgaggctggcctggagtctctgcacgtcctccaccagctgtgcgatctcccgctccttggcggccaactcaacttctaggctggagcgggtcagcacctctatggccacgtctggtgccttctggatctgtgaggccagctggagggagtgattggccgatgagagctgttcccttaaggtctccgcctctctctgagccacctctgccctctggtttgccctttcaaggtccgtcatgatcatttcaatctcgtcggcctttgcagtagtttcttcatcgtatttggttttcaggtcaaataattctgttcgagttttttccagggctgtttgtaggctctgaaccttatgctcagcttcctccagctttgaggtggtggacatctgtgtctcctgcagctttctctccttttctgcaaagtcattctgtaacttctgttccttctcaagagctatggtttcggcttggttcttcagtgtctgttcatattctcggattttctctttaagtgcttttatcgtaacctcttgatttttcacttcagcaaattccttgttgtattcttccagagtttccctaagtttctggttctctgtttcaatatcgtgcaggcgctgcactttgagctggagttgctgtccgagatccaaagctggtacgggatctgggacgtcaatcaatcttttgtagacattcaagaaagctgcttcagcttccttgcttcttttactcagtgcatcaatctctccttggaaactcttcagcagcggcgctacctgcttgcgcaaatcctctggagtgttcttcttgaactcccggctctgttcgataagccgctttctggactgctcactttcatcctgccggttcgccaataccgttgcggtggcatcgagttctctcttcaacctggctccggctacgcacaacatccacctggcagagtcccggggctgtcccggcgccgcgggcgccgagctggcacgtgcggggcggaccctaagggtgcgccgctcctccgggcggggggtggcaggcaggcactcgccccttgggcacggcggcgactcgggcgcgggccggggagccccggcacggtccccccgcggcgccggggactccgcgcgcggaccaccgcccggcatgccacggtcccaacgggcccccggggctctgctttcgagaacccggcccgagaaggcatctccgagcgcacccgccgcgcgctccatggcgggccctgcagagagggcagaagccccgaggggacgcaaggaagggacccggcgccgcaggtcaccgggggccgccggagcccccaggcgcgcggcgatcgcggctcggaccggcggcggggaggcagcgtacactgcccgggcacccgggggaacagcttggggcctgcctaggggaaagttgcagcctcctcctcccgcgcccgcacccggcggtccgggacaccgggacccagcgacactgcgcgcggggcaccc

SEQ ID NO: 9619 - RNA, 3840 nt, Homo sapiens
  source 1..3840: mol_type = other RNA
atcatgatgggctcctcggtgtcggcgctgcctgggccctcagtggcctccacgccgtcgcagctgtcgccctccgagctgggcgccgcccggccgctgcgggccgagggtgagtcgctggcgcccgcctggccctgactcccggcctgaatttcctcaatgaacagttctctgcggatccgagacctgtagttgtggaaccagttgatgacggtgctggttttcaggttgagctgggtggcgaggtcttcgatggtttttggtgacgggtatggcttttgctgatacgctcgtttcagcgcctccttctcctccggagccagcaccacccggggtttcttcagctggtgctggggctgggggctggcgccctggctgtactcggtgccgacagagggcggttcgcagggctggctgtcactgactgagctgtgccgccgcttcatgtaggctttcttctccatccgtttcatgtccatcagcttctccacattgttggggtcgttcagccacagctgcatccggacgaagggctctcgtcctttcagactgagcttatgccagggtttggggcgggcaaggaggtcagagacagagccttgggtgagccctaagatggtctccccaaataagcgctggccgaggttgttgtccgtcagcacctccttcacccgcttggttatgccgtaggtgtccagctccggggacatggctactaattcttggatgctgagggccgagtgtccggagagaggcagcggggttgtgggctgggagtcggatgctggcgggtcactgggctctggtggcttgctgtccttgctcgcctcgatggggggacagggctgctggaccagctcggtcaggctcttcaccgactcactggaactcatcggggactcaggggcagggctgcagctggcggaggtctttggagtgctttctgagctcacacagccctgctgcagcgggtcctggagcgatgtcacggagtggaggactggcccttgctgctggccctggacgggtagaacaccctggcctagctcgccgttcagccagagctgcatccggatgaagggttctcggcctttctgcgtcagcttgctccatggcttcggtcgggacagcatgtcgctgacgctgccctgggacaggcccagcaccttctccccgaagattctctggcagatgccgttcttggccagcttttccttaacctgccgggtgagctcgatggtgtccacctcctggtacatgtagacctcgtactgctcgggggtcagcggggggaccgagggcttggtgggcttggacatgggcacgatcggggaggatggcagggggctgttctgtggtgtctcgctgcggctggccccggtcagactcagctctgagctctgggagtatggggactcagcgctgggccactccttccagtactctgacgacgagggtccctggagctgactgcgctcggcccgaggctggctgccacctccgctgccaccgctgcccttctctttcccgccgcccgtttcttcggccttggcctcctcggaggaggcggcatttcttctctccggctgcaccgcgctccaccagtggtccttccaggcaccgctgcggcccacctcatttttcacctgtctcaggaccccttgtgcacaatcggctgctccctgggggtccagcccgggggcgtcctgggcctcctttttgagggccggggggttcggcagagcagaggcaccggcctcaggagctgcggagggcttcttcagggagatggcgagaggtgggtagctggacacggtgggcatgggcgaggtggacagaagcttgggggtgaggatggtgatgtcactctgggacagtggtgcctgctttaaggcagggtcgagggcagcctgctgggcctccatctcccggcgggcttgctgcaggatggagcggatggcgtcatcagagttcccgctgccggatgcggaggaaggctgggccggctctgcagttttctgcacttggagctccctcttggcttgctctaggatggacttgatggcttcatcagagccagtctccgaggctcggatccgggtggtgatgttaccttcagacccatttcttcgtttcggtacttcctgaaatagtctgttcaggctctggcctggattctctctttgtctgccttggatgctacggagggccaggatgttctgctcatcggagaggaactgtttcatcttgtgaaatggctccttgccacgaacagtcagtttattccatggcttgggccgggccagaatctcgctcacggacccttgagacagtcccaacacataatgtccgaaaatacgttgtccgatattgtgcttaatcagctgctctttgacctgccgggcgatttctgcagtgtccatctcctcgccctcggagacgctcccagcactttctgactggctgggggatggggccatgccattgacatctgggctttgttgtaatggactttgggaagatatggagtttgtgctgtatggaccgctcaggtcgctgttggagatgcgcagcgcggcgttctcggactgcagcgagcggttcttctccagcaacagcacctccaggggcttggccgcatcctgtgtcccagcgccctcggacggtgcaaactccatggacttcagaatgttcagctctttcttcacctcttcatagtcagcctggcctttgagtttttcttccagttgtttgagtgtgctgtttttggcgctcagctgctgctcaagctgtgagatctggctggccgaattctcccgcagcttggtgaggctggcctggagtctctgcacgtcctccaccagctgtgcgatctcccgctccttggcggccaactcaacttctaggctggagcgggtcagcacctctatggcctgctccacgtctggtgccttctggatctgtgaggccagctggagggagtgattggccgatgagagctgttcccttaaggtctccgcctctctctgagccacctctgccctctggtttgccctttcaaggtccgtcatgatcatttcaatctcgtcggcctttgcagtagtttcttcatcgtatttggttttcaggtcaaataattctgttcgagttttttccagggctgtttgtaggctctgaaccttatgctcagcttcctccagctttgaggtggtggacatctgtgtctcctgcagctttctctccttttctgcaaagtcattctgtaacttctgttccttctcaagagctatggtttcggcttggttcttcagtgtctgttcatattctcggattttctctttaagtgcttttatcgtaacctcttgatttttcacttcagcaaattccttgttgtattcttccagagtttccctaagtttctggttctctgtttcaatatcgtgcaggcgctgcactttgagctggagttgctgtccgagatccaaagctggtacgggatctgggacgtcaatcaatcttttgtagacattcaagaaagctgcttcagcttccttgcttcttttactcagtgcatcaatctctccttggaaactcttcagcagcggcgctacctgcttgcgcaaatcctctggagtgttcttcttgaactcccggctctgttcgataagccgctttctggactgctcactttcatcctgccggttcgccaataccgttgcggtggcatcgagttctctctgcagctgctgtaaatcaaagcgcttccaatattgaaacatcgatcccacattggccgccatcttgagacatattgagacggagtgagcggctgatagagag

SEQ ID NO: 9620 - RNA, 4130 nt, Homo sapiens
  source 1..4130: mol_type = other RNA
atcatgatgggctcctcggtgtcggcgctgcctgggccctcagtggcctccacgccgtcgcagctgtcgccctccgagctgggcgccgcccggccgctgcgggccgagggtgagtcgctggcgcccgcctggccctgactcccggcctgaatttcctcaatgaacagttctctgcggatccgagacctgtagttgtggaaccagttgatgacggtgctggttttcaggttgagctgggtggcgaggtcttcgatggtttttggtgacgggtatggcttttgctgatacgctcgtttcagcgcctccttctcctccggagccagcaccacccggggtttcttcagctggtgctggggctgggggctggcgccctggctgtactcggtgccgacagagggcggttcgcagggctggctgtcactgactgagctgtgccgccgcttcatgtaggctttcttctccatccgtttcatgtccatcagcttctccacattgttggggtcgttcagccacagctgcatccggacgaagggctctcgtcctttcagactgagcttatgccagggtttggggcgggcaaggaggtcagagacagagccttgggtgagccctaagatggtctccccaaataagcgctggccgaggttgttgtccgtcagcacctccttcacccgcttggttatgccgtaggtgtccagctccggggacatggctactaattcttggatgctgagggccgagtgtccggagagaggcagcggggttgtgggctgggagtcggatgctggcgggtcactgggctctggtggcttgctgtccttgctcgcctcgatggggggacagggctgctggaccagctcggtcaggctcttcaccgactcactggaactcatcggggactcaggggcagggctgcagctggcggaggtctttggagtgctttctgagctcacacagccctgctgcagcgggtcctggagcgatgtcacggagtggaggactggcccttgctgctggccctggacgggtagaacaccctggcctagctcgccgttcagccagagctgcatccggatgaagggttctcggcctttctgcgtcagcttgctccatggcttcggtcgggacagcatgtcgctgacgctgccctgggacaggcccagcaccttctccccgaagattctctggcagatgccgttcttggccagcttttccttaacctgccgggtgagctcgatggtgtccacctcctggtacatgtagacctcgtactgctcgggggtcagcggggggaccgagggcttggtgggcttggacatgggcacgatcggggaggatggcagggggctgttctgtggtgtctcgctgcggctggccccggtcagactcagctctgagctctgggagtatggggactcagcgctgggccactccttccagtactctgacgacgagggtccctggagctgactgcgctcggcccgaggctggctgccacctccgctgccaccgctgcccttctctttcccgccgcccgtttcttcggccttggcctcctcggaggaggcggcatttcttctctccggctgcaccgcgctccaccagtggtccttccaggcaccgctgcggcccacctcatttttcacctgtctcaggaccccttgtgcacaatcggctgctccctgggggtccagcccgggggcgtcctgggcctcctttttgagggccggggggttcggcagagcagaggcaccggcctcaggagctgcggagggcttcttcagggagatggcgagaggtgggtagctggacacggtgggcatgggcgaggtggacagaagcttgggggtgaggatggtgatgtcactctgggacagtggtgcctgctttaaggcagggtcgagggcagcctgctgggcctccatctcccggcgggcttgctgcaggatggagcggatggcgtcatcagagttcccgctgccggatgcggaggaaggctgggccggctctgcagttttctgcacttggagctccctcttggcttgctctaggatggacttgatggcttcatcagagccagtctccgaggctcggatccgggtggtgatgttaccttcagacccatttcttcgtttcggtacttcctgaaatagtctgttcaggctctggcctggattctctctttgtctgccttggatgctacggagggccaggatgttctgctcatcggagaggaactgtttcatcttgtgaaatggctccttgccacgaacagtcagtttattccatggcttgggccgggccagaatctcgctcacggacccttgagacagtcccaacacataatgtccgaaaatacgttgtccgatattgtgcttaatcagctgctctttgacctgccgggcgatttctgcagtgtccatctcctcgccctcggagacgctcccagcactttctgactggctgggggatggggccatgccattgacatctgggctttgttgtaatggactttgggaagatatggagtttgtgctgtatggacctgttgaaaaaatcatgcttgtgcttccggcttcctgcatagccttggagtagaaggactgcattagctgccgctggagaagagagtttagtgcaaattttcctgtagaagccaggggtaggctggggcttgccagggatgagctgaaaaagtcttgacttaaccccgctggtgagaactggtgtgtaccattagtattggaagcctgctcccccgggttgcggggcaactgagaaggagggggggccggcaaagatcccgggcgccgactttcaggctggtctttccctttcctcctggctgacccgctcaggtcgctgttggagatgcgcagcgcggcgttctcggactgcagcgagcggttcttctccagcaacagcacctccaggggcttggccgcatcctgtgtcccagcgccctcggacggtgcaaactccatggacttcagaatgttcagctctttcttcacctcttcatagtcagcctggcctttgagtttttcttccagttgtttgagtgtgctgtttttggcgctcagctgctgctcaagctgtgagatctggctggccgaattctcccgcagcttggtgaggctggcctggagtctctgcacgtcctccaccagctgtgcgatctcccgctccttggcggccaactcaacttctaggctggagcgggtcagcacctctatggcctgctccacgtctggtgccttctggatctgtgaggccagctggagggagtgattggccgatgagagctgttcccttaaggtctccgcctctctctgagccacctctgccctctggtttgccctttcaaggtccgtcatgatcatttcaatctcgtcggcctttgcagtagtttcttcatcgtatttggttttcaggtcaaataattctgttcgagttttttccagggctgtttgtaggctctgaaccttatgctcagcttcctccagctttgaggtggtggacatctgtgtctcctgcagctttctctccttttctgcaaagtcattctgtaacttctgttccttctcaagagctatggtttcggcttggttcttcagtgtctgttcatattctcggattttctctttaagtgcttttatcgtaacctcttgatttttcacttcagcaaattccttgttgtattcttccagagtttccctaagtttctggttctctgtttcaatatcgtgcaggcgctgcactttgagctggagttgctgtccgagatccaaagctggtacgggatctgggacgtcaatcaatcttttgtagacattcaagaaagctgcttcagcttccttgcttcttttactcagtgcatcaatctctccttggaaactcttcagcagcggcgctacctgcttgcgcaaatcctctggagtgttcttcttgaactcccggctctgttcgataagccgctttctggactgctcactttcatcctgccggttcgccaataccgttgcggtggcatcgagttctctctgcagctgctgtaaatcaaagcgcttccaatattgaaacatcgatcccacattggccgccatcttgagacatattgagacggagtg

SEQ ID NO: 9621 - RNA, 4087 nt, Homo sapiens
  source 1..4087: mol_type = other RNA
atcatgatgggctcctcggtgtcggcgctgcctgggccctcagtggcctccacgccgtcgcagctgtcgccctccgagctgggcgccgcccggccgctgcgggccgagggtgagtcgctggcgcccgcctggccctgactcccggcctgaatttcctcaatgaacagttctctgcggatccgagacctgtagttgtggaaccagttgatgacggtgctggttttcaggttgagctgggtggcgaggtcttcgatggtttttggtgacgggtatggcttttgctgatacgctcgtttcagcgcctccttctcctccggagccagcaccacccggggtttcttcagctggtgctggggctgggggctggcgccctggctgtactcggtgccgacagagggcggttcgcagggctggctgtcactgactgagctgtgccgccgcttcatgtaggctttcttctccatccgtttcatgtccatcagcttctccacattgttggggtcgttcagccacagctgcatccggacgaagggctctcgtcctttcagactgagcttatgccagggtttggggcgggcaaggaggtcagagacagagccttgggtgagccctaagatggtctccccaaataagcgctggccgaggttgttgtccgtcagcacctccttcacccgcttggttatgccgtaggtgtccagctccggggacatggctactaattcttggatgctgagggccgagtgtccggagagaggcagcggggttgtgggctgggagtcggatgctggcgggtcactgggctctggtggcttgctgtccttgctcgcctcgatggggggacagggctgctggaccagctcggtcaggctcttcaccgactcactggaactcatcggggactcaggggcagggctgcagctggcggaggtctttggagtgctttctgagctcacacagccctgctgcagcgggtcctggagcgatgtcacggagtggaggactggcccttgctgctggccctggacgggtagaacaccctggcctagctcgccgttcagccagagctgcatccggatgaagggttctcggcctttctgcgtcagcttgctccatggcttcggtcgggacagcatgtcgctgacgctgccctgggacaggcccagcaccttctccccgaagattctctggcagatgccgttcttggccagcttttccttaacctgccgggtgagctcgatggtgtccacctcctggtacatgtagacctcgtactgctcgggggtcagcggggggaccgagggcttggtgggcttggacatgggcacgatcggggaggatggcagggggctgttctgtggtgtctcgctgcggctggccccggtcagactcagctctgagctctgggagtatggggactcagcgctgggccactccttccagtactctgacgacgagggtccctggagctgactgcgctcggcccgaggctggctgccacctccgctgccaccgctgcccttctctttcccgccgcccgtttcttcggccttggcctcctcggaggaggcggcatttcttctctccggctgcaccgcgctccaccagtggtccttccaggcaccgctgcggcccacctcatttttcacctgtctcaggaccccttgtgcacaatcggctgctccctgggggtccagcccgggggcgtcctgggcctcctttttgagggccggggggttcggcagagcagaggcaccggcctcaggagctgcggagggcttcttcagggagatggcgagaggtgggtagctggacacggtgggcatgggcgaggtggacagaagcttgggggtgaggatggtgatgtcactctgggacagtggtgcctgctttaaggcagggtcgagggcagcctgctgggcctccatctcccggcgggcttgctgcaggatggagcggatggcgtcatcagagttcccgctgccggatgcggaggaaggctgggccggctctgcagttttctgcacttggagctccctcttggcttgctctaggatggacttgatggcttcatcagagccagtctccgaggctcggatccgggtggtgatgttaccttcagacccatttcttcgtttcggtacttcctgaaatagtctgttcaggctctggcctggattctctctttgtctgccttggatgctacggagggccaggatgttctgctcatcggagaggaactgtttcatcttgtgaaatggctccttgccacgaacagtcagtttattccatggcttgggccgggccagaatctcgctcacggacccttgagacagtcccaacacataatgtccgaaaatacgttgtccgatattgtgcttaatcagctgctctttgacctgccgggcgatttctgcagtgtccatctcctcgccctcggagacgctcccagcactttctgactggctgggggatggggccatgccattgacatctgggctttgttgtaatggactttgggaagatatggagtttgtgctgtatggacctgttgaaaaaatcatgcttgtgcttccggcttcctgcatagccttggagtagaaggactgcattagctgccgctggagaagagagtttagtgcaaattttcctgtagaagccaggggtaggctggggcttgccagggatgagctgaaaaagtcttgacttaaccccgctggtgagaactggtgtgtaccattagtattggaagcctgctcccccgggttgcggggcaactgagaaggagggggggccggcaaagatcccgggcgccgactttcaggctggtctttccctttcctcctggctgacccgctcaggtcgctgttggagatgcgcagcgcggcgttctcggactgcagcgagcggttcttctccagcaacagcacctccaggggcttggccgcatcctgtgtcccagcgccctcggacggtgcaaactccatggacttcagaatgttcagctctttcttcacctcttcatagtcagcctggcctttgagtttttcttccagttgtttgagtgtgctgtttttggcgctcagctgctgctcaagctgtgagatctggctggccgaattctcccgcagcttggtgaggctggcctggagtctctgcacgtcctccaccagctgtgcgatctcccgctccttggcggccaactcaacttctaggctggagcgggtcagcacctctatggcctgctccacgtctggtgccttctggatctgtgaggccagctggagggagtgattggccgatgagagctgttcccttaaggtctccgcctctctctgagccacctctgccctctggtttgccctttcaaggtccgtcatgatcatttcaatctcgtcggcctttgcagtagtttcttcatcgtatttggttttcaggtcaaataattctgttcgagttttttccagggctgtttgtaggctctgaaccttatgctcagcttcctccagctttgaggtggtggacatctgtgtctcctgcagctttctctccttttctgcaaagtcattctgtaacttctgttccttctcaagagctatggtttcggcttggttcttcagtgtctgttcatattctcggattttctctttaagtgcttttatcgtaacctcttgatttttcacttcagcaaattccttgttgtattcttccagagtttccctaagtttctggttctctgtttcaatatcgtgcaggcgctgcactttgagctggagttgctgtccgagatccaaagctggtacgggatctgggacgtcaatcaatcttttgtagacattcaagaaagctgcttcagcttccttgcttcttttactcagtgcatcaatctctccttggaaactcttcagcagcggcgctacctgcttgcgcaaatcctctggagtgttcttcttgaactcccggctctgttcgataagccgctttctggactgctcactttcatcctgccggttcgccaataccgttgcggtggcatcgagttctctcttcaacctggctccggctacgcacaacatccacctggcagagt

SEQ ID NO: 9622 - RNA, 3202 nt, Homo sapiens
  source 1..3202: mol_type = other RNA
atcatgatgggctcctcggtgttctccaggtagcggcaccacaccatgaaggcagcccgtattggaagaatcttcatctccgcttgagagtactcaacctcgataggggagatgttgcgggagtagaaagcgcagcaggctctcttgccggtttggtcgtcgatttggatcagggaggcgtgcagggccgtgccggtgacgccggtttccaagtagaatgggttctggggcttggggtggtggaggagaggcgccttgcggaaagccctcttcaggcactcgaaggcctcttgctcctcgactccccagtagaactggtaggagctcagcagctgccgcaccaggggctctgcgatgatgctgaagcgctccacgaagtggcggtaggggaagacgaattcgatgaagtttcgcagagatagcttggagccaggggtagggtaccctgttatgatggtcatgacgttcttgttcagtttcacccctttgggggtgacgacgaagcccaggaattccacggtttggcggtggaactggctcttgtccagggagcagtagacgttgtgatggcggaagcggaccaggacttggcggacgtggtggaggtgctcctcctgactcattgagtagatcaggacttcctggccataagaaagcacaaagaaccctagcatgtcctttaggatgaagtgaatcacgttctgaggtatgatagggtctggggagagcgcaaacggctggtagctcttcatctcttcaagctccaaaccaaacgctgctttccacacatcttcggtgcggtgcccgttcacgctttcctccacaatggtcccacgcagctccagttttgtgaaccactcggctccgtgtaactggtcaaacagttccggaatcatctgtatgtagtcctgtctgttggtcagcatgtcctgcaggtcccagtattcctcctgtagcctggctctttcttgcatcctggcacccacaggttcccaaggcgcggtggagggacactcgtaaaaggtctcgctgtgatcactgtctccagcctgctgaagctcagagggctctgattcagaaagatcatcggatccgtctgagcttggctggtcggaagtctcatcatctgcttccttcgggttaaacacgtcggccaggtctgagtatgggtgtggcagtccgggtagcaggctcatgccgtgcctctctagggcaatgcatggcgggggcgggcggaagcagttcttcaggcagtagggagagtggaaggtgcagcggcctttgatccagtcgacttcgggggcgtggactcggagccagcggatgcctaggaccacagagaagttcggtgaaggtacgatgtcaaattcgatggactcctggtggttctggtggatacacaccaggggctccgtgtagagccagacaggctcgttgccaatcagcgagccgtccacggattggaccggctgtgggtacggcttctcgtagagctcgacgtagtgctcttgggcgaacttctcatccatgaagttgccgtcagctcccgaatccaccagggcctggaccgcgacgctgtggtaggggttcactctcaccatgagcagcaggaagaggtgggcgcgattgatgtccggatggacttcgctgggcaaccagctgctgaccatccacctctctggagcaggtgagtcgatccaggtcaggttccgggggcgggcctcggggggcagcctgagcatagctcttctctctgccagcttctcttctatttgcaggatgagcacaatcagactgtctagggaatccggctgagggacccggaatagatagtgcctgatctcctcgttgagcccctggcacaagtgggcctgcaggacttcatctggccagcccaagatgggtaccaggctctggaactcatcgatgtactcagtggcagagcggccgccctgcctgatggtgaacatggcctcttctgccacacgcagtgcctggcggtactcaaacacttcggacatggcctccaggaaggctgggaagtctccgatcagggggctgttttcctgcagtagagctttggcccattctaatgccaagccggacaggtgattgatgacatagccaactctcagacggtcgttatagaacattcttgggtagctctgtaaggtcagttggcagagtacgatgaactcgtggaattctctgcgatcgccagagaagtgctttggggcgggcagttggcctgcattgatccctttgatcaagatctcttctgctactctctgttgctctttgaggtcttgcattcggaagtacagcgagatgatggacctcaccatggccataagttctgcggttgagtgctcggtctggttttgctcttgaggagtctcctcccttcccgattccttcaggtcagtgtgagcctcttgttcttctcgggctcccgatgggttgactgatgcttctttcatcctatcagatgctccactgagtggatccccccttgcctggtgtgaaccgttgcatgactcctccaggtcttggagtaggtcattgggtggatcctctatttccttacgtgggccactggatggctcctccatgtcttggagtagatcagtgggcagctcttccatttcctggagtgggccactggggggctccttcttttcctgggctgggccgctggctggccctgcctctccccgcactccactgcccgacgtcgcctcggtggtgttggatgagccctcggaggactccatttgttttgatgatggattcttatgctccatcatcgtctcaaatgagtcttcagagggttctatcatttcgtcggatggaaaggagtgtattctgaagattggtaaggttgtgatggcgtccagtcagtagctgggaccgtggagatcagaaccttggctgcaagcgttcaagtggatctcctcccgtcctgtgccactcgatcctcgctgcttgcttccccgggcccagtcccaagcgtgaggctggggatgaagtgatgccggtggcttagtgatgccggtggcttcctgtcctcgaagctcagtcggtcgtctctcagctggtgtgaggctgggccaggatggaaccccagactctccgaggctccccaccacaccctgctgctgaaggctgctcagcgaggctgtgccgagtgctgggggggtgt

SEQ ID NO: 9623 - RNA, 4442 nt, Homo sapiens
  source 1..4442: mol_type = other RNA
atcatgatgggctcctcggtgttttcgtgtctggctctttcgtgttttaacattgtggtaaatcgagtgtaggaggccgggcacctgcctttgcaggagctgatgaggtggcggtggtggtggtggtggtgatggtggtggtggtggctggatccgtaaaagctttcggaggatgtgaaggaaaagtgatcaaagtcactttcactgcagaaggatgacccctctaggtgaatgtagtcactgtggtcggacacaaccccgtcctggtcgctgtcggaaaactccacgtgtgctcggggctgctcatcgctggtgacttcaatgtgaatgggcaccagggcgttagactggcagcctcgccggccccgagcgggggggccgctttgattttcttcctccagcaaatactcaatggaaaaccgcctcttgggacataggccattttgcggtggttctagggttacgggagacagcatgtcatcccctaaatttggcatggatttggacttctggatcagcttttcgaattcggagatgcgtgtgggcaccatgtcccggggcacctcctccgtggagcactggctccaggcgcgcagcaggtccttgtgctgctgctcgctctcgtactgcagaatcctggacttcacggagcagatcacctcggagttcatcaggtccttgcggttgatgcggtgcattttcttgtacatcttcaggaaccccggggcgttgcgggctgacctgtgtctgatccttgatctgccgttactgcgaacctccgggacgtagggggacccccacgccatggggcagctctccttggagtcctcctcacataacagggagcccatgctttccgacttgactttcgggtccgggaagctatcgcagtcgtcgtttaggagatcgtcacagctccgggatttgattttgggagagacggtttcttccgtgctgctccagatttctgcgttttgccgggccatttgccagccgttcttgaaactaatggctcttggtgagtcccgagggacatccaagtgctgtctgtaagtgctacagtaatctaactcactggaggggttgccgttgagccctgagtaactgcaaagggatggacatattttgctatcatccccaccttttgctcttgatggggaagaaggagaagagctagtgaaagactttgtaagagtggtgcttgatcctgggaggtccactcggcctgggctagtcctgctcgcactttgatctcccaagccccgtggtggacccactgcaggctcgctcttcctccgcttcctgaagtcactggccatgcttgcagaactcatgggtctttccaggcttctgtctatagaggactgatacaaggaggcctcattgaaaacaccagaagaatgatcttgaacatagtccagaggctttttaggaggcgggcgtccaaactccagttctgaaaagaatttataccagggctcattttctaaatctatgtcatctggatttatgcgatcagtccgggtgggagacagagccggggcgcgcgagcttggtgtgggggcgccactccggggcggaggggaggggctaccagtgacttctccgagtcgggagctagaaagaggcttccggccaggttcccttggaacaggtgtcggagttgttgggagagggggtggtctttcatgctgaagaattgatgacttgccaggttcatattcaaaaatactccttggctcagaccgaaattttcttgtgtccacttttctgtctggaggatcccagtcatgcttttctgttgaagaccgatctcttggtcgaagcggcgggactggaggtggaacatgtgggggaggcactggggaggacgcatccttaaaggcattggggctgttgtcggagtggcttttggaaagaggtctgtaggtttgggtctttgcagcagggtgtgactgagcactgtagggtgggttgtacagacctgcattgtatgtataaggagtattatacatgtctgtgtcatcatccggcttgtgcaccatgtgaatttgcttaaacatcgtcttgtaccagtccttgggccggtcgactgtcgttctaattgctgtggggattccggattcatccacgggcccgatccctgggtaatgcggggctttgatgactgtcactctcttctcttcctctgaggatcggtacagggggatagagctgctggtggtgccatccagagactgcgcatgctggggatatgtgtctgtggaatcgagggatgtgccgtgctgcatgacaatgctggagttgagtgaggctgggagagaatatgccgagggggaaaacggcctctgatagtaactcatgggactcacggcacctcctgagtttccattcactgttatctggctatgagtggccgcaggggtggttaaggtggtgccatctgtcacagcagacctctgaccccaggtgggggagggtgtctcagaacggccagtggtgtcagagtcaccaatctgcagctcctccagcatggctgtggaggactcactctccgagcgggaggagtgctcggccagggaggagtctgttgtcagagagcctgtgtcgtggctgtggatgaggctttctggagctgggagcaggtgtttgtataagcaatgggaaaggctctggggattatgcaggcgtgaagaccccacaccatcggggggcggaaggctgagtgatgctgagctggtgccactgcctggtgagaaagtggctcggttcaaaggtaccacggaaggagggcacggaggagaagcttctggtgtggtttgtctgtgtgtctgtgaagcatttacctccaacacactggcaggtaagttctgatttccaagcactctgcagtctgaggactgagaggccgctgcaactgcagatttttgtctctcttgctgaagaggtatctttgcagtctctggagaaagctcaggtagctgtttgtggctttcaagatcctgtcctgaaaggggagctatctgaatggaaagagatgctgtgtgtgtctcaggcactggattaggggtcagtgagcggggccttttgagaaatgacggtacttcgacagatttggagaactgtggagtactaatggggctgctacttcctagatcctggttatgggttagtttcaaggtagaaatcctccgagtttgagaatcttgcctgtagtcctcttgtagaactggggtgttgatgttagcgaatggtgcaggatccgtgctggaagctgctggtagtggattagtgattttttgtgtatatgacatggttgtgttagattcttcagaatatacaattgtctgtctcgaatcttcattggaatacatagttccctgaagaggttttttgttagcaaagtactctgtactggagggaatttgtgtgttagttactaactggtctaaaatgacaccctttgtgtgactggttatcaaagagctatgaaagctctcttttctttctggtggagggggtgcctgagttggtgatcttttatcttgtaggtttggtcgaacgcttctaaaaccttttgctgagtctggtgactgagaatcacgccctgcagccaataggtttggagaactttgcactctcttcacagatgttagcgtaacagacatggcggcacgtttgcgagcacacccaccgctatctgtgttcattttcaccttggagagtttgttattaaagtcttcagttttcctacaggcagctgagttcaacagttgctctatacagaggaagtaggagtcagtggccttttacatgtagagattgtttatttagccctttttaaaaggtcttgaactccagaggtttaagattaagtccaatccaagtgtctctgtcagtgtactgggacgctcaggaagccccttctccgcctcggcctcagcgtgcagacatatgccctgggagcccacaatctgttaacaggaagcaggtaaacccgagagcgtccgcctgcgttccagtccagtgcccgtcccagcacacacctgctttttcagacctgccgctcatatgccacagccacgcacaggaccagcgttagcagagtgcaacaccctccgtttggatccctcgttttcagggtaagcagctagggagctgctgagataatattgcagggaaagcttgccttcccaagacaaaaacctttgctgctgcctgatagcagatatgcagcattatcactctgcattccacattctccaatcagctaattggaacggcagtcaacagcctgtccaaaaggcagcttgcaggcctgcgtggctgtgatcattgtatactaacatgcccattgcttctctcttccctgaagagatgtataaaagaggcttcttccagggcgaagctcagcagaatatgccacactgttttccataagt

SEQ ID NO: 9624 - RNA, 4507 nt, Homo sapiens
  source 1..4507: mol_type = other RNA
atcatgatgggctcctcggtgttttcgtgtctggctctttcgtgttttaacattgtggtaaatcgagtgtaggaggccgggcacctgcctttgcaggagctgatgaggtggcggtggtggtggtggtggtgatggtggtggtggtggctggatccgtaaaagctttcggaggatgtgaaggaaaagtgatcaaagtcactttcactgcagaaggatgacccctctaggtgaatgtagtcactgtggtcggacacaaccccgtcctggtcgctgtcggaaaactccacgtgtgctcggggctgctcatcgctggtgacttcaatgtgaatgggcaccagggcgttagactggcagcctcgccggccccgagcgggggggccgctttgattttcttcctccagcaaatactcaatggaaaaccgcctcttgggacataggccattttgcggtggttctagggttacgggagacagcatgtcatcccctaaatttggcatggatttggacttctggatcagcttttcgaattcggagatgcgtgtgggcaccatgtcccggggcacctcctccgtggagcactggctccaggcgcgcagcaggtccttgtgctgctgctcgctctcgtactgcagaatcctggacttcacggagcagatcacctcggagttcatcaggtccttgcggttgatgcggtgcattttcttgtacatcttcaggaaccccggggcgttgcgggctgacctgtgtctgatccttgatctgccgttactgcgaacctccgggacgtagggggacccccacgccatggggcagctctccttggagtcctcctcacataacagggagcccatgctttccgacttgactttcgggtccgggaagctatcgcagtcgtcgtttaggagatcgtcacagctccgggatttgattttgggagagacggtttcttccgtgctgctccagatttctgcgttttgccgggccatttgccagccgttcttgaaactaatggctcttggtgagtcccgagggacatccaagtgctgtctgtaagtgctacagtaatctaactcactggaggggttgccgttgagccctgagtaactgcaaagggatggacatattttgctatcatccccaccttttgctcttgatggggaagaaggagaagagctagtgaaagactttgtaagagtggtgcttgatcctgggaggtccactcggcctgggctagtcctgctcgcactttgatctcccaagccccgtggtggacccactgcaggctcgctcttcctccgcttcctgaagtcactggccatgcttgcagaactcatgggtctttccaggcttctgtctatagaggactgatacaaggaggcctcattgaaaacaccagaagaatgatcttgaacatagtccagaggctttttaggaggcgggcgtccaaactccagttctgaaaagaatttataccagggctcattttctaaatctatgtcatctggatttatgcgatcagtccgggtgggagacagagccggggcgcgcgagcttggtgtgggggcgccactccggggcggaggggaggggctaccagtgacttctccgagtcgggagctagaaagaggcttccggccaggttcccttggaacaggtgtcggagttgttgggagagggggtggtctttcatgctgaagaattgatgacttgccaggttcatattcaaaaatactccttggctcagaccgaaattttcttgtgtccacttttctgtctggaggatcccagtcatgcttttctgttgaagaccgatctcttggtcgaagcggcgggactggaggtggaacatgtgggggaggcactggggaggacgcatccttaaaggcattggggctgttgtcggagtggcttttggaaagaggtctgtaggtttgggtctttgcagcagggtgtgactgagcactgtagggtgggttgtacagacctgcattgtatgtataaggagtattatacatgtctgtgtcatcatccggcttgtgcaccatgtgaatttgcttaaacatcgtcttgtaccagtccttgggccggtcgactgtcgttctaattgctgtggggattccggattcatccacgggcccgatccctgggtaatgcggggctttgatgactgtcactctcttctcttcctctgaggatcggtacagggggatagagctgctggtggtgccatccagagactgcgcatgctggggatatgtgtctgtggaatcgagggatgtgccgtgctgcatgacaatgctggagttgagtgaggctgggagagaatatgccgagggggaaaacggcctctgatagtaactcatgggactcacggcacctcctgagtttccattcactgttatctggctatgagtggccgcaggggtggttaaggtggtgccatctgtcacagcagacctctgaccccaggtgggggagggtgtctcagaacggccagtggtgtcagagtcaccaatctgcagctcctccagcatggctgtggaggactcactctccgagcgggaggagtgctcggccagggaggagtctgttgtcagagagcctgtgtcgtggctgtggatgaggctttctggagctgggagcaggtgtttgtataagcaatgggaaaggctctggggattatgcaggcgtgaagaccccacaccatcggggggcggaaggctgagtgatgctgagctggtgccactgcctggtgagaaagtggctcggttcaaaggtaccacggaaggagggcacggaggagaagcttctggtgtggtttgtctgtgtgtctgtgaagcatttacctccaacacactggcaggtaagttctgatttccaagcactctgcagtctgaggactgagaggccgctgcaactgcagatttttgtctctcttgctgaagaggtatctttgcagtctctggagaaagctcaggtagctgtttgtggctttcaagatcctgtcctgaaaggggagctatctgaatggaaagagatgctgtgtgtgtctcaggcactggattaggggtcagtgagcggggccttttgagaaatgacggtacttcgacagatttggagaactgtggagtactaatggggctgctacttcctagatcctggttatgggttagtttcaaggtagaaatcctccgagtttgagaatcttgcctgtagtcctcttgtagaactggggtgttgatgttagcgaatggtgcaggatccgtgctggaagctgctggtagtggattagtgattttttgtgtatatgacatggttgtgttagattcttcagaatatacaattgtctgtctcgaatcttcattggaatacatagttccctgaagaggttttttgttagcaaagtactctgtactggagggaatttgtgtgttagttactaactggtctaaaatgacaccctttgtgtgactggttatcaaagagctatgaaagctctcttttctttctggtggagggggtgcctgagttggtgatcttttatcttgtaggtttggtcgaacgcttctaaaaccttttgctgcaagagaggaatatgtagcatctccgttcagtgtctcctgattgccatcattgtaagatctccaagctgagtctggtgactgagaatcacgccctgcagccaataggtttggagaactttgcactctcttcacagatgttagcgtaacagacatggcggcacgtttgcgagcacacccaccgctatctgtgttcattttcaccttggagagtttgttattaaagtcttcagttttcaggcagctgagttcaacagttgctctatacagaggaagtaggagtcagtggccttttacatgtagagattgtttatttagccctttttaaaaggtcttgaactccagaggtttaagattaagtccaatccaagtgtctctgtcagtgtactgggacgctcaggaagccccttctccgcctcggcctcagcgtgcagacatatgccctgggagcccacaatctgttaacaggaagcaggtaaacccgagagcgtccgcctgcgttccagtccagtgcccgtcccagcacacacctgctttttcagacctgccgctcatatgccacagccacgcacaggaccagcgttagcagagtgcaacaccctccgtttggatccctcgttttcagggtaagcagctagggagctgctgagataatattgcagggaaagcttgccttcccaagacaaaaacctttgctgctgcctgatagcagatatgcagcattatcactctgcattccacattctccaatcagctaattggaacggcagtcaacagcctgtccaaaaggcagcttgcaggcctgcgtggctgtgatcattgtatactaacatgcccattgcttctctcttccctgaagagatgtataaaagaggcttcttccagggcgaagctcagcagaatatgccacactgttttccataagt

SEQ ID NO: 9625 - RNA, 4511 nt, Homo sapiens
  source 1..4511: mol_type = other RNA
atcatgatgggctcctcggtgttttcgtgtctggctctttcgtgttttaacattgtggtaaatcgagtgtaggaggccgggcacctgcctttgcaggagctgatgaggtggcggtggtggtggtggtggtgatggtggtggtggtggctggatccgtaaaagctttcggaggatgtgaaggaaaagtgatcaaagtcactttcactgcagaaggatgacccctctaggtgaatgtagtcactgtggtcggacacaaccccgtcctggtcgctgtcggaaaactccacgtgtgctcggggctgctcatcgctggtgacttcaatgtgaatgggcaccagggcgttagactggcagcctcgccggccccgagcgggggggccgctttgattttcttcctccagcaaatactcaatggaaaaccgcctcttgggacataggccattttgcggtggttctagggttacgggagacagcatgtcatcccctaaatttggcatggatttggacttctggatcagcttttcgaattcggagatgcgtgtgggcaccatgtcccggggcacctcctccgtggagcactggctccaggcgcgcagcaggtccttgtgctgctgctcgctctcgtactgcagaatcctggacttcacggagcagatcacctcggagttcatcaggtccttgcggttgatgcggtgcattttcttgtacatcttcaggaaccccggggcgttgcgggctgacctgtgtctgatccttgatctgccgttactgcgaacctccgggacgtagggggacccccacgccatggggcagctctccttggagtcctcctcacataacagggagcccatgctttccgacttgactttcgggtccgggaagctatcgcagtcgtcgtttaggagatcgtcacagctccgggatttgattttgggagagacggtttcttccgtgctgctccagatttctgcgttttgccgggccatttgccagccgttcttgaaactaatggctcttggtgagtcccgagggacatccaagtgctgtctgtaagtgctacagtaatctaactcactggaggggttgccgttgagccctgagtaactgcaaagggatggacatattttgctatcatccccaccttttgctcttgatggggaagaaggagaagagctagtgaaagactttgtaagagtggtgcttgatcctgggaggtccactcggcctgggctagtcctgctcgcactttgatctcccaagccccgtggtggacccactgcaggctcgctcttcctccgcttcctgaagtcactggccatgcttgcagaactcatgggtctttccaggcttctgtctatagaggactgatacaaggaggcctcattgaaaacaccagaagaatgatcttgaacatagtccagaggctttttaggaggcgggcgtccaaactccagttctgaaaagaatttataccagggctcattttctaaatctatgtcatctggatttatgcgatcagtccgggtgggagacagagccggggcgcgcgagcttggtgtgggggcgccactccggggcggaggggaggggctaccagtgacttctccgagtcgggagctagaaagaggcttccggccaggttcccttggaacaggtgtcggagttgttgggagagggggtggtctttcatgctgaagaattgatgacttgccaggttcatattcaaaaatactccttggctcagaccgaaattttcttgtgtccacttttctgtctggaggatcccagtcatgcttttctgttgaagaccgatctcttggtcgaagcggcgggactggaggtggaacatgtgggggaggcactggggaggacgcatccttaaaggcattggggctgttgtcggagtggcttttggaaagaggtctgtaggtttgggtctttgcagcagggtgtgactgagcactgtagggtgggttgtacagacctgcattgtatgtataaggagtattatacatgtctgtgtcatcatccggcttgtgcaccatgtgaatttgcttaaacatcgtcttgtaccagtccttgggccggtcgactgtcgttctaattgctgtggggattccggattcatccacgggcccgatccctgggtaatgcggggctttgatgactgtcactctcttctcttcctctgaggatcggtacagggggatagagctgctggtggtgccatccagagactgcgcatgctggggatatgtgtctgtggaatcgagggatgtgccgtgctgcatgacaatgctggagttgagtgaggctgggagagaatatgccgagggggaaaacggcctctgatagtaactcatgggactcacggcacctcctgagtttccattcactgttatctggctatgagtggccgcaggggtggttaaggtggtgccatctgtcacagcagacctctgaccccaggtgggggagggtgtctcagaacggccagtggtgtcagagtcaccaatctgcagctcctccagcatggctgtggaggactcactctccgagcgggaggagtgctcggccagggaggagtctgttgtcagagagcctgtgtcgtggctgtggatgaggctttctggagctgggagcaggtgtttgtataagcaatgggaaaggctctggggattatgcaggcgtgaagaccccacaccatcggggggcggaaggctgagtgatgctgagctggtgccactgcctggtgagaaagtggctcggttcaaaggtaccacggaaggagggcacggaggagaagcttctggtgtggtttgtctgtgtgtctgtgaagcatttacctccaacacactggcaggtaagttctgatttccaagcactctgcagtctgaggactgagaggccgctgcaactgcagatttttgtctctcttgctgaagaggtatctttgcagtctctggagaaagctcaggtagctgtttgtggctttcaagatcctgtcctgaaaggggagctatctgaatggaaagagatgctgtgtgtgtctcaggcactggattaggggtcagtgagcggggccttttgagaaatgacggtacttcgacagatttggagaactgtggagtactaatggggctgctacttcctagatcctggttatgggttagtttcaaggtagaaatcctccgagtttgagaatcttgcctgtagtcctcttgtagaactggggtgttgatgttagcgaatggtgcaggatccgtgctggaagctgctggtagtggattagtgattttttgtgtatatgacatggttgtgttagattcttcagaatatacaattgtctgtctcgaatcttcattggaatacatagttccctgaagaggttttttgttagcaaagtactctgtactggagggaatttgtgtgttagttactaactggtctaaaatgacaccctttgtgtgactggttatcaaagagctatgaaagctctcttttctttctggtggagggggtgcctgagttggtgatcttttatcttgtaggtttggtcgaacgcttctaaaaccttttgctgcaagagaggaatatgtagcatctccgttcagtgtctcctgattgccatcattgtaagatctccaagctgagtctggtgactgagaatcacgccctgcagccaataggtttggagaactttgcactctcttcacagatgttagcgtaacagacatggcggcacgtttgcgagcacacccaccgctatctgtgttcattttcaccttggagagtttgttattaaagtcttcagttttcctacaggcagctgagttcaacagttgctctatacagaggaagtaggagtcagtggccttttacatgtagagattgtttatttagccctttttaaaaggtcttgaactccagaggtttaagattaagtccaatccaagtgtctctgtcagtgtactgggacgctcaggaagccccttctccgcctcggcctcagcgtgcagacatatgccctgggagcccacaatctgttaacaggaagcaggtaaacccgagagcgtccgcctgcgttccagtccagtgcccgtcccagcacacacctgctttttcagacctgccgctcatatgccacagccacgcacaggaccagcgttagcagagtgcaacaccctccgtttggatccctcgttttcagggtaagcagctagggagctgctgagataatattgcagggaaagcttgccttcccaagacaaaaacctttgctgctgcctgatagcagatatgcagcattatcactctgcattccacattctccaatcagctaattggaacggcagtcaacagcctgtccaaaaggcagcttgcaggcctgcgtggctgtgatcattgtatactaacatgcccattgcttctctcttccctgaagagatgtataaaagaggcttcttccagggcgaagctcagcagaatatgccacactgttttccataagt

SEQ ID NO: 9626 - RNA, 4567 nt, Homo sapiens
  source 1..4567: mol_type = other RNA
atcatgatgggctcctcggtgttttcgtgtctggctctttcgtgttttaacattgtggtaaatcgagtgtaggaggccgggcacctgcctttgcaggagctgatgaggtggcggtggtggtggtggtggtgatggtggtggtggtggctggatccgtaaaagctttcggaggatgtgaaggaaaagtgatcaaagtcactttcactgcagaaggatgacccctctaggtgaatgtagtcactgtggtcggacacaaccccgtcctggtcgctgtcggaaaactccacgtgtgctcggggctgctcatcgctggtgacttcaatgtgaatgggcaccagggcgttagactggcagcctcgccggccccgagcgggggggccgctttgattttcttcctccagcaaatactcaatggaaaaccgcctcttgggacataggccattttgcggtggttctagggttacgggagacagcatgtcatcccctaaatttggcatggatttggacttctggatcagcttttcgaattcggagatgcgtgtgggcaccatgtcccggggcacctcctccgtggagcactggctccaggcgcgcagcaggtccttgtgctgctgctcgctctcgtactgcagaatcctggacttcacggagcagatcacctcggagttcatcaggtccttgcggttgatgcggtgcattttcttgtacatcttcaggaaccccggggcgttgcgggctgacctgtgtctgatccttgatctgccgttactgcgaacctccgggacgtagggggacccccacgccatggggcagctctccttggagtcctcctcacataacagggagcccatgctttccgacttgactttcgggtccgggaagctatcgcagtcgtcgtttaggagatcgtcacagctccgggatttgattttgggagagacggtttcttccgtgctgctccagatttctgcgttttgccgggccatttgccagccgttcttgaaactaatggctcttggtgagtcccgagggacatccaagtgctgtctgtaagtgctacagtaatctaactcactggaggggttgccgttgagccctgagtaactgcaaagggatggacatattttgctatcatccccaccttttgctcttgatggggaagaaggagaagagctagtgaaagactttgtaagagtggtgcttgatcctgggaggtccactcggcctgggctagtcctgctcgcactttgatctcccaagccccgtggtggacccactgcaggctcgctcttcctccgcttcctgaagtcactggccatgcttgcagaactcatgggtctttccaggcttctgtctatagaggactgatacaaggaggcctcattgaaaacaccagaagaatgatcttgaacatagtccagaggctttttaggaggcgggcgtccaaactccagttctgaaaagaatttataccagggctcattttctaaatctatgtcatctggatttatgcgatcagtccgggtgggagacagagccggggcgcgcgagcttggtgtgggggcgccactccggggcggaggggaggggctaccagtgacttctccgagtcgggagctagaaagaggcttccggccaggttcccttggaacaggtgtcggagttgttgggagagggggtggtctttcatgctgaagaattgatgacttgccaggttcatattcaaaaatactccttggctcagaccgaaattttcttgtgtccacttttctgtctggaggatcccagtcatgcttttctgttgaagaccgatctcttggtcgaagcggcgggactggaggtggaacatgtgggggaggcactggggaggacgcatccttaaaggcattggggctgttgtcggagtggcttttggaaagaggtctgtaggtttgggtctttgcagcagggtgtgactgagcactgtagggtgggttgtacagacctgcattgtatgtataaggagtattatacatgtctgtgtcatcatccggcttgtgcaccatgtgaatttgcttaaacatcgtcttgtaccagtccttgggccggtcgactgtcgttctaattgctgtggggattccggattcatccacgggcccgatccctgggtaatgcggggctttgatgactgtcactctcttctcttcctctgaggatcggtacagggggatagagctgctggtggtgccatccagagactgcgcatgctggggatatgtgtctgtggaatcgagggatgtgccgtgctgcatgacaatgctggagttgagtgaggctgggagagaatatgccgagggggaaaacggcctctgatagtaactcatgggactcacggcacctcctgagtttccattcactgttatctggctatgagtggccgcaggggtggttaaggtggtgccatctgtcacagcagacctctgaccccaggtgggggagggtgtctcagaacggccagtggtgtcagagtcaccaatctgcagctcctccagcatggctgtggaggactcactctccgagcgggaggagtgctcggccagggaggagtctgttgtcagagagcctgtgtcgtggctgtggatgaggctttctggagctgggagcaggtgtttgtataagcaatgggaaaggctctggggattatgcaggcgtgaagaccccacaccatcggggggcggaaggctgagtgatgctgagctggtgccactgcctggtgagaaagtggctcggttcaaaggtaccacggaaggagggcacggaggagaagcttctggtgtggtttgtctgtgtgtctgtgaagcatttacctccaacacactggcaggtaagttctgatttccaagcactctgcagtctgaggactgagaggccgctgcaactgcagatttttgtctctcttgctgaagaggtatctttgcagtctctggagaaagctcaggtagctgtttgtggctttcaagatcctgtcctgaaaggggagctatctgaatggaaagagatgctgtgtgtgtctcaggcactggattaggggtcagtgagcggggccttttgagaaatgacggtacttcgacagatttggagaactgtggagtactaatggggctgctacttcctagatcctggttatgggttagtttcaaggtagaaatcctccgagtttgagaatcttgcctgtagtcctcttgtagaactggggtgttgatgttagcgaatggtgcaggatccgtgctggaagctgctggtagtggattagtgattttttgtgtatatgacatggttgtgttagattcttcagaatatacaattgtctgtctcgaatcttcattggaatacatagttccctgaagaggttttttgttagcaaagtactctgtactggagggaatttgtgtgttagttactaactggtctaaaatgacaccctttgtgtgactggttatcaaagagctatgaaagctctcttttctttctggtggagggggtgcctgagttggtgatcttttatcttgtaggtttggtcgaacgcttctaaaaccttttgctgcaagagaggaatatgtagcatctccgttcagtgtctcctgattgccatcattgtaagatctccaagctgagtctggtgactgagaatcacgccctgcagccaataggtttggagaactttgcactctcttcacagatgttagcgtaacagacatggcggcacgtttgcgagcacacccaccgctatctgtgttcattttcaccttggagagtttgttattaaagtcttcagttttccttctgaagaaatgcacccagatcagaatggtatacgagtctgtcctattctcgctctacaggcagctgagttcaacagttgctctatacagaggaagtaggagtcagtggccttttacatgtagagattgtttatttagccctttttaaaaggtcttgaactccagaggtttaagattaagtccaatccaagtgtctctgtcagtgtactgggacgctcaggaagccccttctccgcctcggcctcagcgtgcagacatatgccctgggagcccacaatctgttaacaggaagcaggtaaacccgagagcgtccgcctgcgttccagtccagtgcccgtcccagcacacacctgctttttcagacctgccgctcatatgccacagccacgcacaggaccagcgttagcagagtgcaacaccctccgtttggatccctcgttttcagggtaagcagctagggagctgctgagataatattgcagggaaagcttgccttcccaagacaaaaacctttgctgctgcctgatagcagatatgcagcattatcactctgcattccacattctccaatcagctaattggaacggcagtcaacagcctgtccaaaaggcagcttgcaggcctgcgtggctgtgatcattgtatactaacatgcccattgcttctctcttccctgaagagatgtataaaagaggcttcttccagggcgaagctcagcagaatatgccacactgttttccataagt

SEQ ID NO: 9627 - RNA, 4474 nt, Homo sapiens
  source 1..4474: mol_type = other RNA
atcatgatgggctcctcggtgttttcgtgtctggctctttcgtgttttaacattgtggtaaatcgagtgtaggaggccgggcacctgcctttgcaggagctgatgaggtggcggtggtggtggtggtggtgatggtggtggtggtggctggatccgtaaaagctttcggaggatgtgaaggaaaagtgatcaaagtcactttcactgcagaaggatgacccctctaggtgaatgtagtcactgtggtcggacacaaccccgtcctggtcgctgtcggaaaactccacgtgtgctcggggctgctcatcgctggtgacttcaatgtgaatgggcaccagggcgttagactggcagcctcgccggccccgagcgggggggccgctttgattttcttcctccagcaaatactcaatggaaaaccgcctcttgggacataggccattttgcggtggttctagggttacgggagacagcatgtcatcccctaaatttggcatggatttggacttctggatcagcttttcgaattcggagatgcgtgtgggcaccatgtcccggggcacctcctccgtggagcactggctccaggcgcgcagcaggtccttgtgctgctgctcgctctcgtactgcagaatcctggacttcacggagcagatcacctcggagttcatcaggtccttgcggttgatgcggtgcattttcttgtacatcttcaggaaccccggggcgttgcgggctgacctgtgtctgatccttgatctgccgttactgcgaacctccgggacgtagggggacccccacgccatggggcagctctccttggagtcctcctcacataacagggagcccatgctttccgacttgactttcgggtccgggaagctatcgcagtcgtcgtttaggagatcgtcacagctccgggatttgattttgggagagacggtttcttccgtgctgctccagatttctgcgttttgccgggccatttgccagccgttcttgaaactaatggctcttggtgagtcccgagggacatccaagtgctgtctgtaagtgctacagtaatctaactcactggaggggttgccgttgagccctgagtaactgcaaagggatggacatattttgctatcatccccaccttttgctcttgatggggaagaaggagaagagctagtgaaagactttgtaagagtggtgcttgatcctgggaggtccactcggcctgggctagtcctgctcgcactttgatctcccaagccccgtggtggacccactgcaggctcgctcttcctccgcttcctgaagtcactggccatgcttgcagaactcatgggtctttccaggcttctgtctatagaggactgatacaaggaggcctcattgaaaacaccagaagaatgatcttgaacatagtccagaggctttttaggaggcgggcgtccaaactccagttctgaaaagaatttataccagggctcattttctaaatctatgtcatctggatttatgcgatcagtccgggtgggagacagagccggggcgcgcgagcttggtgtgggggcgccactccggggcggaggggaggggctaccagtgacttctccgagtcgggagctagaaagaggcttccggccaggttcccttggaacaggtgtcggagttgttgggagagggggtggtctttcatgctgaagaattgatgacttgccaggttcatattcaaaaatactccttggctcagaccgaaattttcttgtgtccacttttctgtctggaggatcccagtcatgcttttctgttgaagaccgatctcttggtcgaagcggcgggactggaggtggaacatgtgggggaggcactggggaggacgcatccttaaaggcattggggctgttgtcggagtggcttttggaaagaggtctgtaggtttgggtctttgcagcagggtgtgactgagcactgtagggtgggttgtacagacctgcattgtatgtataaggagtattatacatgtctgtgtcatcatccggcttgtgcaccatgtgaatttgcttaaacatcgtcttgtaccagtccttgggccggtcgactgtcgttctaattgctgtggggattccggattcatccacgggcccgatccctgggtaatgcggggctttgatgactgtcactctcttctcttcctctgaggatcggtacagggggatagagctgctggtggtgccatccagagactgcgcatgctggggatatgtgtctgtggaatcgagggatgtgccgtgctgcatgacaatgctggagttgagtgaggctgggagagaatatgccgagggggaaaacggcctctgatagtaactcatgggactcacggcacctcctgagtttccattcactgttatctggctatgagtggccgcaggggtggttaaggtggtgccatctgtcacagcagacctctgaccccaggtgggggagggtgtctcagaacggccagtggtgtcagagtcaccaatctgcagctcctccagcatggctgtggaggactcactctccgagcgggaggagtgctcggccagggaggagtctgttgtcagagagcctgtgtcgtggctgtggatgaggctttctggagctgggagcaggtgtttgtataagcaatgggaaaggctctggggattatgcaggcgtgaagaccccacaccatcggggggcggaaggctgagtgatgctgagctggtgccactgcctggtgagaaagtggctcggttcaaaggtaccacggaaggagggcacggaggagaagcttctggtgtggtttgtctgtgtgtctgtgaagcatttacctccaacacactggcaggtaagttctgatttccaagcactctgcagtctgaggactgagaggccgctgcaactgcagatttttgtctctcttgctgaagaggtatctttgcagtctctggagaaagctcaggtagctgtttgtggctttcaagatcctgtcctgaaaggggagctatctgaatggaaagagatgctgtgtgtgtctcaggcactggattaggggtcagtgagcggggccttttgagaaatgacggtacttcgacagatttggagaactgtggagtactaatggggctgctacttcctagatcctggttatgggttagtttcaaggtagaaatcctccgagtttgagaatcttgcctgtagtcctcttgtagaactggggtgttgatgttagcgaatggtgcaggatccgtgctggaagctgctggtagtggattagtgattttttgtgtatatgacatggttgtgttagattcttcagaatatacaattgtctgtctcgaatcttcattggaatacatagttccctgaagaggttttttgttagcaaagtactctgtactggagggaatttgtgtgttagttactaactggtctaaaatgacaccctttgtgtgactggttatcaaagagctatgaaagctctcttttctttctggtggagggggtgcctgagttggtgatcttttatcttgtaggtttggtcgaacgcttctaaaaccttttgctgcaagagaggaatatgtagcatctccgttcagtgtctcctgattgccatcattgtaagatctccaagctgagtctggtgactgagaatcacgccctgtgttcattttcaccttggagagtttgttattaaagtcttcagttttccttctgaagaaatgcacccagatcagaatggtatacgagtctgtcctattctcgctctacaggcagctgagttcaacagttgctctatacagaggaagtaggagtcagtggccttttacatgtagagattgtttatttagccctttttaaaaggtcttgaactccagaggtttaagattaagtccaatccaagtgtctctgtcagtgtactgggacgctcaggaagccccttctccgcctcggcctcagcgtgcagacatatgccctgggagcccacaatctgttaacaggaagcaggtaaacccgagagcgtccgcctgcgttccagtccagtgcccgtcccagcacacacctgctttttcagacctgccgctcatatgccacagccacgcacaggaccagcgttagcagagtgcaacaccctccgtttggatccctcgttttcagggtaagcagctagggagctgctgagataatattgcagggaaagcttgccttcccaagacaaaaacctttgctgctgcctgatagcagatatgcagcattatcactctgcattccacattctccaatcagctaattggaacggcagtcaacagcctgtccaaaaggcagcttgcaggcctgcgtggctgtgatcattgtatactaacatgcccattgcttctctcttccctgaagagatgtataaaagaggcttcttccagggcgaagctcagcagaatatgccacactgttttccataagt

SEQ ID NO: 9628 - RNA, 1883 nt, Homo sapiens
  source 1..1883: mol_type = other RNA
atcatgatgggctcctcggtgttttcgtgtctggctctttcgtgttttaacattgtggtaaatcgagtgtaggaggccgggcacctgcctttgcaggagctgatgaggtggcggtggtggtggtggtggtgatggtggtggtggtggctggatccgtaaaagctttcggaggatgtgaaggaaaagtgatcaaagtcactttcactgcagaaggatgacccctctaggtgaatgtagtcactgtggtcggacacaaccccgtcctggtcgctgtcggaaaactccacgtgtgctcggggctgctcatcgctggtgacttcaatgtgaatgggcaccagggcgttagactggcagcctcgccggccccgagcgggggggccgctttgattttcttcctccagcaaatactcaatggaaaaccgcctcttgggacataggccattttgcggtggttctagggttacgggagacagcatgtcatcccctaaatttggcatggatttggacttctggatcagcttttcgaattcggagatgcgtgtgggcaccatgtcccggggcacctcctccgtggagcactggctccaggcgcgcagcaggtccttgtgctgctgctcgctctcgtactgcagaatcctggacttcacggagcagatcacctcggagttcatcaggtccttgcggttgatgcggtgcattttcttgtacatcttcaggaaccccggggcgttgcgggctgacctgtgtctgatccttgatctgccgttactgcgaacctccgggacgtagggggacccccacgccatggggcagctctccttggagtcctcctcacataacagggagcccatgctttccgacttgactttcgggtccgggaagctatcgcagtcgtcgtttaggagatcgtcacagctccgggatttgattttgggagagacggtttcttccgtgctgctccagatttctgcgttttgccgggccatttgccagccgttcttgaaactaatggctcttggtgagtcccgagggacatccaagtgctgtctgtaagtgctacagtaatctaactcactggaggggttgccgttgagccctgagtaactgcaaagggatggacatattttgctatcatccccaccttttgctcttgatggggaagaaggagaagagctagtgaaagactttgtaagagtggtgcttgatcctgggaggtccactcggcctgggctagtcctgctcgcactttgatctcccaagccccgtggtggacccactgcaggctcgctcttcctccgcttcctgaagtcactggccatgcttgcagaactcatgggtctttccaggcttctgtctatagaggactgatacaaggaggctggtctttcatgctgaagaattgatgacttgccaggttcatattcaaaaatactccttggctcagaccgaaattttcttgtgtccacttttctgtctggaggatcccagtcatgcttttctgttgaagaccgatctcttggtcgaagcggcgggactggaggtggaacatgtgggggaggcactggggaggacgcatccttaaaggcattggggctgttgtcggagtggcttttggaaagaggtctgtaggtttgggtctttgcagcagggtgtgactgagcactgtagggtgggttgtacagacccggcttgtgcaccatgtgaatttgcttaaacatcgtcttgtaccagtccttgggccggtcgactgtctgcaaaggtgttgttgctttcatcctgtccccggcttccttctcccggctggcacaagccttctcttccagtggacttggtcagccagctgctgcctgcccaggctctcagaagctgcctctgctactgct

SEQ ID NO: 9629 - RNA, 2577 nt, Homo sapiens
  source 1..2577: mol_type = other RNA
atcatgatgggctcctcggtgttttcgtgtctggctctttcgtgttttaacattgtggtaaatcgagtgtaggaggccgggcacctgcctttgcaggagctgatgaggtggcggtggtggtggtggtggtgatggtggtggtggtggctggatccgtaaaagctttcggaggatgtgaaggaaaagtgatcaaagtcactttcactgcagaaggatgacccctctaggtgaatgtagtcactgtggtcggacacaaccccgtcctggtcgctgtcggaaaactccacgtgtgctcggggctgctcatcgctggtgacttcaatgtgaatgggcaccagggcgttagactggcagcctcgccggccccgagcgggggggccgctttgattttcttcctccagcaaatactcaatggaaaaccgcctcttgggacataggccattttgcggtggttctagggttacgggagacagcatgtcatcccctaaatttggcatggatttggacttctggatcagcttttcgaattcggagatgcgtgtgggcaccatgtcccggggcacctcctccgtggagcactggctccaggcgcgcagcaggtccttgtgctgctgctcgctctcgtactgcagaatcctggacttcacggagcagatcacctcggagttcatcaggtccttgcggttgatgcggtgcattttcttgtacatcttcaggaaccccggggcgttgcgggctgacctgtgtctgatccttgatctgccgttactgcgaacctccgggacgtagggggacccccacgccatggggcagctctccttggagtcctcctcacataacagggagcccatgctttccgacttgactttcgggtccgggaagctatcgcagtcgtcgtttaggagatcgtcacagctccgggatttgattttgggagagacggtttcttccgtgctgctccagatttctgcgttttgccgggccatttgccagccgttcttgaaactaatggctcttggtgagtcccgagggacatccaagtgctgtctgtaagtgctacagtaatctaactcactggaggggttgccgttgagccctgagtaactgcaaagggatggacatattttgctatcatccccaccttttgctcttgatggggaagaaggagaagagctagtgaaagactttgtaagagtggtgcttgatcctgggaggtccactcggcctgggctagtcctgctcgcactttgatctcccaagccccgtggtggacccactgcaggctcgctcttcctccgcttcctgaagtcactggccatgcttgcagaactcatgggtctttccaggcttctgtctatagaggactgatacaaggaggctggtctttcatgctgaagaattgatgacttgccaggttcatattcaaaaatactccttggctcagaccgaaattttcttgtgtccacttttctgtctggaggatcccagtcatgcttttctgttgaagaccgatctcttggtcgaagcggcgggactggaggtggaacatgtgggggaggcactggggaggacgcatccttaaaggcattggggctgttgtcggagtggcttttggaaagaggtctgtaggtttgggtctttgcagcagggtgtgactgagcactgtagggtgggttgtacagacctgcattgtatgtataaggagtattatacatgtctgtgtcatcatccggcttgtgcaccatgtgaatttgcttaaacatcgtcttgtaccagtccttgggccggtcgactgtcgttctaattgctgtggggattccggattcatccacgggcccgatccctgggtaatgcggggctttgatgactgtcactctcttctcttcctctgaggatcggtacagggggatagagctgctggtggtgccatccagagactgcgcatgctggggatatgtgtctgtggaatcgagggatgtgccgtgctgcatgacaatgctggagttgagtgaggctgggagagaatatgccgagggggaaaacggcctctgatagtaactcatgggactcacggcacctcctgagtttccattcactgttatctggctctgagttggtgatcttttatcttgtaggtttggtcgaacgcttctaaaaccttttgctgcaagagaggaatatgtagcatctccgttcagtgtctcctgattgccatcattgtaagatctccaagctgagtctggtgactgagaatcacgccctacaggcagctgagttcaacagttgctctatacagaggaagtaggagtcagtggccttttacatgtagagattgtttatttagccctttttaaaaggtcttgaactccagaggtttaagattaagtccaatccaagtgtctttggatgggcacattccagcacaggaaaatcgctgtcttgtcggctgctgtgcagaatgagttgcttgggcaggtattcctctattctcagctcccgggtctgccttgtagccgcagccagcctagggagcatttacggcatgtacgtggtgttcatccacaataaaaggagact

SEQ ID NO: 9630 - RNA, 2797 nt, Homo sapiens
  source 1..2797: mol_type = other RNA
atcatgatgggctcctcggtgttttcgtgtctggctctttcgtgttttaacattgtggtaaatcgagtgtaggaggccgggcacctgcctttgcaggagctgatgaggtggcggtggtggtggtggtggtgatggtggtggtggtggctggatccgtaaaagctttcggaggatgtgaaggaaaagtgatcaaagtcactttcactgcagaaggatgacccctctaggtgaatgtagtcactgtggtcggacacaaccccgtcctggtcgctgtcggaaaactccacgtgtgctcggggctgctcatcgctggtgacttcaatgtgaatgggcaccagggcgttagactggcagcctcgccggccccgagcgggggggccgctttgattttcttcctccagcaaatactcaatggaaaaccgcctcttgggacataggccattttgcggtggttctagggttacgggagacagcatgtcatcccctaaatttggcatggatttggacttctggatcagcttttcgaattcggagatgcgtgtgggcaccatgtcccggggcacctcctccgtggagcactggctccaggcgcgcagcaggtccttgtgctgctgctcgctctcgtactgcagaatcctggacttcacggagcagatcacctcggagttcatcaggtccttgcggttgatgcggtgcattttcttgtacatcttcaggaaccccggggcgttgcgggctgacctgtgtctgatccttgatctgccgttactgcgaacctccgggacgtagggggacccccacgccatggggcagctctccttggagtcctcctcacataacagggagcccatgctttccgacttgactttcgggtccgggaagctatcgcagtcgtcgtttaggagatcgtcacagctccgggatttgattttgggagagacggtttcttccgtgctgctccagatttctgcgttttgccgggccatttgccagccgttcttgaaactaatggctcttggtgagtcccgagggacatccaagtgctgtctgtaagtgctacagtaatctaactcactggaggggttgccgttgagccctgagtaactgcaaagggatggacatattttgctatcatccccaccttttgctcttgatggggaagaaggagaagagctagtgaaagactttgtaagagtggtgcttgatcctgggaggtccactcggcctgggctagtcctgctcgcactttgatctcccaagccccgtggtggacccactgcaggctcgctcttcctccgcttcctgaagtcactggccatgcttgcagaactcatgggtctttccaggcttctgtctatagaggactgatacaaggaggctggtctttcatgctgaagaattgatgacttgccaggttcatattcaaaaatactccttggctcagaccgaaattttcttgtgtccacttttctgtctggaggatcccagtcatgcttttctgttgaagaccgatctcttggtcgaagcggcgggactggaggtggaacatgtgggggaggcactggggaggacgcatccttaaaggcattggggctgttgtcggagtggcttttggaaagaggtctgtaggtttgggtctttgcagcagggtgtgactgagcactgtagggtgggttgtacagacctgcattgtatgtataaggagtattatacatgtctgtgtcatcatccggcttgtgcaccatgtgaatttgcttaaacatcgtcttgtaccagtccttgggccggtcgactgtcgttctaattgctgtggggattccggattcatccacgggcccgatccctgggtaatgcggggctttgatgactgtcactctcttctcttcctctgaggatcggtacagggggatagagctgctggtggtgccatccagagactgcgcatgctggggatatgtgtctgtggaatcgagggatgtgccgtgctgcatgacaatgctggagttgagtgaggctgggagagaatatgccgagggggaaaacggcctctgatagtaactcatgggactcacggcacctcctgagtttccattcactgttatctggctctgagttggtgatcttttatcttgtaggtttggtcgaacgcttctaaaaccttttgctgcaagagaggaatatgtagcatctccgttcagtgtctcctgattgccatcattgtaagatctccaagctgagtctggtgactgagaatcacgccctgcagccaataggtttggagaactttgcactctcttcacagatgttagcgtaacagacatggcggcacgtttgcgagcacacccaccgctatctgtgttcattttcaccttggagagtttgttattaaagtcttcagttttcctacaggcagctgagttcaacagttgctctatacagaggaagtaggagtcagtggccttttacatgtagagattgtttatttagccctttttaaaaggtcttgaactccagaggtttaagattaagtccaatccaagtgtcaggtgcttcatggcccccagggaacttgcagaacatcaaaattagattttgactgattttccaacaaattggttggctttggatgggcacattccagcacaggaaaatcgctgtcttgtcggctgctgtgcagaatgagttgcttgggcaggtattcctctattctcagctcccgggtctgccttgtagccgcagccagcctagggagcatttacggcatgtacgtggtgttcatccacaataaaaggagact

SEQ ID NO: 9631 - RNA, 550 nt, Homo sapiens
  source 1..550: mol_type = other RNA
atcccaccactgccaccatctgcccaaggcccttcctcttcattcttcaagccgaaagcacagctgatatgttgggtgatgtttcttgacagctgtcttgccgaggatgtatgtgattcagaactgttgttactatagctctgctcatctgggtcttgtttctttgagtctttggctccttccaaaagatcactgagaacctgtatatattcagtcgcacctttaaggatatcaactttgctgggcttcctgctttggggaagaaatggcacaagtgccttcaatctggcaaaaccacggttgagattttttatccgctcacgctccttggcgttggccacacgccgccgctccagcaccaactggaggttttcagtggacgagtagccgcccgagggcagccgcttgagccggcagacagcggccagctggggcagcggcccgaactgctcccgcaacacgtcctccagcacctcggcttgcggggtgcccaggagcgcgggcggcgcggcgcggggatctaggacgccgggcgcggggtccatggcag

SEQ ID NO: 9632 - RNA, 2548 nt, Homo sapiens
  source 1..2548: mol_type = other RNA
atcccaccactgccaccatgccaacccctcatccccaaagagacccaaacagtgcagaggtgcatcaatcaacctttaatgtccaaaagaggcgtggatgcagagcataggagatgtggcagggtctcaggccctgctccagaaatgagggagagatgaacacaaaccagacactttcaactggccacacagtctgggagggcagggggaaacacagatttggacattcataaaaaaataaaacctaaaatcaagcactcaattttgtgcccactgaagggtttgataaagggaactcagtcaccacccaggtctcccctcccctgccaacatcacaaagcaagctcggcacacactaagggcttagggaggggtattctcctgcctccccaccagccccaagaatggacttgaaaataaaagaataagctggatcccccacccccccacattgtcaaccctacacgagagttttgaaggcgactcatgaaaatcagcagctcaaacggcaatgaccaccccaccccaaaccccaccccactcctatttcattaacagacaagatttcccctgcatcctcctcagaatctcctcctctcacagccctgctccatctcctatgtcctggcttcaccactgcaagactgacctcctccaaggctcccagaagctcctcttagctctttatcacttctatcctcacctcccaccagagactgcaaccatccacagtcactgtccctctgcactgagacccagctccagagcagatggcagcatggtcatcctgtcctgggtggtcctcctaaagccttcccagggagcagacagccagagagcaagcagagtgtctgggctagatgacagcaaggaggggacacctatctttattttcaaaacagatatccccagaggcttttagcataaaagcccacttagaactaactgtgccccctacctacccatacaccctagagattccacactgtcctgccccctccctcccttctaccccaaaccccacacacacatacacacacatatacacacatattcacacatatacacagaagagtcaagggagacatcaatttggtttgattgctaagacctaactaaggaactacagtcaccagaaattcccttgccagccaactaacaacaggggctgctctaagagaactccagaggaatgaggaaactgagggctaagcagggagcagacaggagaaaaatgtaaagaaaaaaaagattcaagctaatcctaccccagcatcctcctgtcatgatctctggcaggaagaacaaaagaaggtaatccacaaagacacagcccttacttagaaattctgacaaagacagcaagacaaatctgctccccactcccacacaccacagacaaacacatctcagggcccctaaagaaggcatccccaccccaccctccgccccaagccatagaatcacagttcagtggaatattctccctggtactagatcaatccctccaccttccttcctacccctttttccttgacaatcccaacactgtccccctgcagcctccctggccctcccaaagcagcatccaccgccaggaagaggcagctgcacagttttagttccacctccagagacctatttcttttcctcagccctcctagtctttcggccgcctagtctctatggtgggccttttattttgtatagggaaagaaagagaaaagggagaggtgggagagatttcctagtgcaatacaaccaaaaaatatttttaaagtcttgaaaaataaacataaagcagccttcttcccccaggcaactaaacagaaagaggtttggttttgtttactgcgacatacacatgaaatcgagtatacagtccatgcagtagcacagccattggagaggacatcctgatgctggctccagtgcaaaacagtcccagcaacgccgcctgcttgccatcgctgccgccgccactgacaccttcaccatggccacctagcctgacttgaagaggaggattgcaacttgacccaagtaaaaatagatgaagtgctttgtctcgtgtgtgacgtagctgccaaaatttcggcccacgatacaatgccaggtagggttatatttcttgtcaaattccttcttgatataggcagcaatgtccttctctatattgtacttctccatggcctgcgtggcgcagtcaacggcatcctgttgcatgtcctcagacatgtctgcgttcttgatcactgccttccggtcagacatggtgtgacacttcacggaggcgagtccgcactgggccctggggaggagcgatggcccgaggcagagcacaggcaggggcggtgttccctgggctcctcctgcagctgcagcagccgccgccgccgcggtctccggctcccgcagcccgaggccgatcgctccctgccgcggtccgcccttggagtttcgccggccgcccgcgctccgcctcacgccgcccgcccgcccgcccgctccgcactggcgcctcacagctccgctccgctctgccgct

SEQ ID NO: 9633 - RNA, 536 nt, Homo sapiens
  source 1..536: mol_type = other RNA
atcccaccactgccaccatggggcacctgaggaacgggaggggtgtgatactgcgagtgcggagacgcgagtccgttcccaggggtgttgctcatcattctgttcggctgatccatcagatgcatcttttgttgttcatactgattatagtgatcaaaatgtgtcagctttgtttgattttgattagttgaaggatgatgaagggatggctgtaaagaggcaaagccttggtctattggcatttgctgacccataggatttactggattttccgggtaaccacattctccgaggccttcaagaccttcactgaaaatattcccatcctcgccaaaaagactcatcattcctggatctgccatcttcttccaacacacggctcctccaaaccacagctcaggagcttgcctgtgcttcacttcactgaggtgtttgccctcaaagcctataatccttaactaatcttcttcatgtcattccatatttctttaattctcttggaccctgcagtgtcaggcaaagtctggatataggtc

SEQ ID NO: 9634 - RNA, 929 nt, Homo sapiens
  source 1..929: mol_type = other RNA
atcccaccactgccaccatggggcacctgaggaacgggaggggtgtgatactgcgagtgcggagacgcgagtccgttcccaggggtgttgctcatcattctgttcggctgatccatcagatgcatcttttgttgttcatactgattatagtgatcaaaatgtgtcagctttgtttgattttgattagttgaaggatgatgaagggatggctgtaaagaggcaaagccttggtctattggcatttgctgacccataggatttactggattttccgggtaaccacattctccgaggccttcaagaccttcactgaaaatattcccatcctcgccaaaaagactcatcattcctggatctgccatcttcttccaacacacggctcctccaaaccacagctcaggagcttgcctgtgcttcacttcactgaggtgtttgccctcaaagcctataatccttaactaatcttcttcatgtcattccatatttctttaattctcttggaccctgcagtgtcaggcaaagtctggatataggtccgcttggcctccagccacctcggccgttcacgctccaagccgcggctctctgcgagggcagagcgcacccgggtcacctcgggggccacctggtgaccaccccccaccggcgctgacccccggcgggttggggggcgggggagccgagttgcgttggaaggttaaagtcgctattatgcagctgccgccgccggcggcccggccagctcgacaaggtggggtcccctcctcgccgcgcctcccggcgctcgccccggccccgctccctttcttctcctcctagcgcacttgggagccgccggggagccccaggagcccccaactccgggctcgcaactccgcgcccgcgaccggcactggctgagctcgggacgcctcccgcgccgcgtgttc

SEQ ID NO: 9635 - RNA, 875 nt, Homo sapiens
  source 1..875: mol_type = other RNA
atcccaccactgccaccatggggcacctgaggaacgggaggggtgtgatactgcgagtgcggagacgcgagtccgttcccaggggtgttgctcatcattctgttcggctgatccatcagatgcatcttttgttgttcatactgattatagtgatcaaaatgtgtcagctttgtttgattttgattagttgaaggatgatgaagggatggctgtaaagaggcaaagccttggtctattggcatttgctgacccataggatttactggattttccgggtaaccacattctccgaggccttcaagaccttcactgaaaatattcccatcctcgccaaaaagactcatcattcctggatctgccatcttcttccaacacacggctcctccaaaccacagctcaggagcttgcctgtgcttcacttcactgaggtgtttgccctcaaagcctataatccttaactaatcttcttcatgtcattccatatttctttaattctcttggaccctgcagtgtcaggcaaagtctggatataggtccgggtcggtcgggctcctccgctgcctagtgccgaggggaaaacaaaacgcagagcgggctccggagttggctcggcagctgcggccagggggctgaatccacgggcacggagttggccgggggcgaacgggtctctggtgagtttcagggtgtccgggtccccgggccgcctcctccgcggcgctcctttgtgtaatttcactcgattcaagtttaatccgatagttcccgagcacgagcgcgtccgcaccaccacgactcaacccccgcgccgccgccgccgccgccgctgccgccgccgccgccgccgccgccgcggccccagcacgccagcgcct

SEQ ID NO: 9636 - RNA, 879 nt, Homo sapiens
  source 1..879: mol_type = other RNA
atcccaccactgccaccatggggcacctgaggaacgggaggggtgtgatactgcgagtgcggagacgcgagtccgttcccaggggtgttgctcatcattctgttcggctgatccatcagatgcatcttttgttgttcatactgattatagtgatcaaaatgtgtcagctttgtttgattttgattagttgaaggatgatgaagggatggctgtaaagaggcaaagccttggtctattggcatttgctgacccataggatttactggattttccgggtaaccacattctccgaggccttcaagaccttcactgaaaatattcccatcctcgccaaaaagactcatcattcctggatctgccatcttcttccaacacacggctcctccaaaccacagctcaggagcttgcctgtgcttcacttcactgaggtgtttgccctcaaagcctataatccttaactaatcttcttcatgtcattccatatttctttaattctcttggaccctgcagtgtcaggcaaagtctggatataggtccgggtcggtcgggctcctccgctgcctagtgccgaggggaaaacaaaacgcagagcgggctccggagttggctcggcagctgcggccagggggctgaatccacgggcacggagttggccgggggcgaacgggtctctggtgagtttcagggtgtccgggtccccgggccgcctcctccgcggcgctcctttgtgtaatttcactcgattcaagtttaatccgatagttcccgagcacgagcgcgtccgcaccaccacgactcaacccccgcgccgccgccgccgccgccgctgccgccgccgccgccgccgccgccgcggccccagcacgccagcgcctgcgc

SEQ ID NO: 9637 - RNA, 661 nt, Homo sapiens
  source 1..661: mol_type = other RNA
atcccaccactgccaccatggggcacctgaggaacgggaggggtgtgatactgcgagtgcggagacgcgagtccgttcccaggggtgttgctcatcattctgttcggctgatccatcagatgcatcttttgttgttcatactgattatagtgatcaaaatgtgtcagctttgtttgattttgattagttgaaggatgatgaagggatggctgtaaagaggcaaagccttggtctattggcatttgctgacccataggatttactggattttccgggtaaccacattctccgaggccttcaagaccttcactgaaaatattcccatcctcgccaaaaagactcatcattcctggatctgccatcttcttccaacacacggctcctccaaaccacagctcaggagcttgcctgtgcttcacttcactgaggtgtttgccctcaaagcctataatccttaactaatcttcttcatgtcattccatatttctttaattctcttggaccctgcagtgtcaggcaaagtctggatataggtcctcgctcggtggcggtccccgcgcgggctggcgccgccgcgccgggaggaacgcactttgttcgcgccggtgcggccgcagctcccggcgagcgcggcgtggtcggtccggagcggggggcgggg

SEQ ID NO: 9638 - RNA, 4255 nt, Homo sapiens
  source 1..4255: mol_type = other RNA
atcccaccactgccaccatgttattgctgccagaaattgatggggccacatgaacttgcagactgtaaaataactctgtagctccagctgagttgatggccacgcatttatatatgccagcatctgagatctgggcactttcaatatcaatgatctgtcctctgttcaagaaagtcatgctggtggaacctgagagtagacgattatctttgtaccatgtaataacaggcacaggatttccagctgccttacactccagctgtacagggttgctcaccaacacagtctcattcagcatttttccagcatcttccagactaggtggttcatgaacatgcagttgaatgtgctgttgtgtttctccagctgcgttggtagccacacatgtgtatctgccagcatcttccaacagggttttggcaatttgtagaactcgaccagaagactgtattttaaggtttccttgggcagtgttcacaggctggtcatcttttaaccatgtaatggaaggatttggaatcccattggctatgcactgcaaggcgacaggcttgtattttaccacaactctctcagaaaggcctgaggacttgattgttggaggaacatgaacagtcacttcaaattccttcttgtggtctccagcagtatttgctgccatgcaccgataaaggcctgtgtttgacacttgagcctgagcaataaccagtttgcgtccatttaataaaatcttgaatccatccctttcatcaattaactggccatccttcagccacatgatagttggtgggggagagcctgtcacatgacaatctagctccagtaagttattaaccatcacaatgaagtaagatgtttcatctcctccttctatagctggtggcaccaagacatcaacttcatatttgatttccttttctcctgccacactggtagccacgcatatgtactgtcctcgatcaatttcttgggcactcatgatttcgagtttcttcccaccagcttctatgcggatattgtcattagctttcacaggtacaccatctttcaaccaggtgagaatgggagaagggtttccagcagctttgcactccagtgtcagagaatgagcaataactacttgcttattcaaaggcgtggccaagttgccttcaatcattggaggaacatagacatccacatggaatgatttttcagcagttccagcaacattggctacatgacacgtatatgttgctgaatcagagacctgtgctcgaggaatatgaagatattgtcctttatcaatataaagtgcttgtgagctggacatgattggctgcccgtccttataccaagtaatggcaggcattggaagtccccgtgtttcacattccagtttaataaggctgttgatcaatactgatatgtctgtggtgacatttcctcctttaatactaggtggaatatagatagtcagttttatatccttggcttgtttgccagctgcattagacacagtacattggtagcgccccttgtcatttctccgtgcattctttaaatgtaagacttgtcctctgtctagaagttcaacattaggatcgcccaaaaataaaggcttgccatctttgaaccaatgaatatcaggaaagggagtgcctttgacctggcattcaagggcgacgtcacggttgaggacaactgagacttcatttgggaagttggtacctattatggtgggtggaactagcacatcaatgttaaagtacttctgagaagtgcctgcaatattaattgctttgcaggaatatcttcctgcatcctctggagtggctctgaagagcttcagtatcttcccattgttcacagtctgaatagtgctgctttcagtcacctggacattatctttataccacataatgatgggagatggagtgccttccacttcacagaagagattggtcagctgatttaacaacaccgacacatttgtaacttgttctttatctttaattactggaggaacatggactttgaggttatattttctttctgtggttccagcttcattgactgccacacagatgtactccccattgtcatagggtgtaacagaagcaataaccagcaatgtgccatcttccaagatagaaatgccaggctctctgcctgtcaactctctaccattgtgtaaccatttgatggttggtttaggggtaccttttgcaggacatggaaattcaatgcgttgattggccactctttcttggaaagtagtgttatatggaggttctagatcttccactgtgggtggttcttggacatgtagcgttatctctgtttcatcagtgcctgctatgttagtagcaacacatgtatatatgccagcatctgagggcgtggcttggtcgatgcttaaagttccgtctggattgctaacatggtgctctccatcaaccagcatagtgcttccacctttggaccaggtgattacaggaagaggagtcccttgagcattacatggaatatccactctttgaccaacttggactttgagatgtttaggtccacgctgtatctttggaggaacatggacatttaatttgacagcctgagtcacattcccagcaatatttgtggcaacacaaagatacatcccactatctgaagtgcgggtttcagtgatcttcattgaaccagaagggaggaatgtgtgtcttggagagaacggtgagatgagctgggtttctttggcccaagtaattatgggtggaggtaagctcttcacttcacatggaagtgttacctcttcccctgcaaggacggagatctcaacaggcttatcctgggacagtcctcgttgatctccaaacactctgggccttacatagactgttagctgcactttccttttggcgtagccggctgtattggtggcagtgcagacatactccccactctcctctcctccaggtgataccacatacagactaccatcagctcctgctgaaaacttagcactgctggttgaaatcagctctcctttcttggaccagatgacagacggtttgggatttccacttgctttgcatggtaaagttactggaatgccttcaattgtactgagtatctgctgcccatgctgaatggttggcagaacatgcacaaccacagaggtagttttgttattggtcccagcaacgttactggccacacaagtatattcaccaccatcctgaagctgaactctttcaatatggaggctcccatcactgcgcacagtgatgtaaggattttggagcaacatagctgaattcttaatccaccgacgttctggaatgggatttccagctaacagagtacagggcaaagtaagctgctgtccttcaataacattggccactgaagggctgattccaataagtggagcaacaagtccggtcactgttactgttgtctctgactggatctttccaaactggttttcagcttcacaaatataggttcctttatcacttgcccataagtttaaaataaagagagctcctgttcttagttggctgatggaactaactgaaaaaggtcttgagaaaattggcatgttgtctaatcttcgccatttgattgttggttctggataaccctgaacataacaaggtaatgtcacatttgagccaatttccatagacacatcagcaggttcttgtatgaaaactggaggtgagccaacatccagagttatcttgccagttgctcttccagcctcattgatggctacacaggtataatcgccagcatccagatcttgtgtttcttgaatcttcaaaagtcccaagagagggtcaataatgaggaatgttgagggcctcaactcaagatctcctttgaaccatttaacttgaggtggaggaataccagaggttttgcattccataacggttatatccccaagggcaaccaagagctcactctgaactaccatcaacttaggggcttcaatgtatctgagagtagaattctgtttatctgttccagctgaattacttgctaggcaaccatagatccctgcatctttgggagctgcatttttgataaataaggtaccatctgaggtcatcctatacccagtacctgtgtgaacccacgataaacatatcgttaacggtccaggcaatctttggtttgggataacctgttgcagaacacatgatggagacctcagaccctcctgtgaaagactgattcttgggcatcacagtgactttgggtggtt

SEQ ID NO: 9639 - RNA, 6323 nt, Homo sapiens
  source 1..6323: mol_type = other RNA
atcccaccactgccaccatgttattgctgccagaaattgatggggccacatgaacttgcagactgtaaaataactctgtagctccagctgagttgatggccacgcatttatatatgccagcatctgagatctgggcactttcaatatcaatgatctgtcctctgttcaagaaagtcatgctggtggaacctgagagtagacgattatctttgtaccatgtaataacaggcacaggatttccagctgccttacactccagctgtacagggttgctcaccaacacagtctcattcagcatttttccagcatcttccagactaggtggttcatgaacatgcagttgaatgtgctgttgtgtttctccagctgcgttggtagccacacatgtgtatctgccagcatcttccaacagggttttggcaatttgtagaactcgaccagaagactgtattttaaggtttccttgggcagtgttcacaggctggtcatcttttaaccatgtaatggaaggatttggaatcccattggctatgcactgcaaggcgacaggcttgtattttaccacaactctctcagaaaggcctgaggacttgattgttggaggaacatgaacagtcacttcaaattccttcttgtggtctccagcagtatttgctgccatgcaccgataaaggcctgtgtttgacacttgagcctgagcaataaccagtttgcgtccatttaataaaatcttgaatccatccctttcatcaattaactggccatccttcagccacatgatagttggtgggggagagcctgtcacatgacaatctagctccagtaagttattaaccatcacaatgaagtaagatgtttcatctcctccttctatagctggtggcaccaagacatcaacttcatatttgatttccttttctcctgccacactggtagccacgcatatgtactgtcctcgatcaatttcttgggcactcatgatttcgagtttcttcccaccagcttctatgcggatattgtcattagctttcacaggtacaccatctttcaaccaggtgagaatgggagaagggtttccagcagctttgcactccagtgtcagagaatgagcaataactacttgcttattcaaaggcgtggccaagttgccttcaatcattggaggaacatagacatccacatggaatgatttttcagcagttccagcaacattggctacatgacacgtatatgttgctgaatcagagacctgtgctcgaggaatatgaagatattgtcctttatcaatataaagtgcttgtgagctggacatgattggctgcccgtccttataccaagtaatggcaggcattggaagtccccgtgtttcacattccagtttaataaggctgttgatcaatactgatatgtctgtggtgacatttcctcctttaatactaggtggaatatagatagtcagttttatatccttggcttgtttgccagctgcattagacacagtacattggtagcgccccttgtcatttctccgtgcattctttaaatgtaagacttgtcctctgtctagaagttcaacattaggatcgcccaaaaataaaggcttgccatctttgaaccaatgaatatcaggaaagggagtgcctttgacctggcattcaagggcgacgtcacggttgaggacaactgagacttcatttgggaagttggtacctattatggtgggtggaactagcacatcaatgttaaagtacttctgagaagtgcctgcaatattaattgctttgcaggaatatcttcctgcatcctctggagtggctctgaagagcttcagtatcttcccattgttcacagtctgaatagtgctgctttcagtcacctggacattatctttataccacataatgatgggagatggagtgccttccacttcacagaagagattggtcagctgatttaacaacaccgacacatttgtaacttgttctttatctttaattactggaggaacatggactttgaggttatattttctttctgtggttccagcttcattgactgccacacagatgtactccccattgtcatagggtgtaacagaagcaataaccagcaatgtgccatcttccaagatagaaatgccaggctctctgcctgtcaactctctaccattgtgtaaccatttgatggttggtttaggggtaccttttgcaggacatggaaattcaatgcgttgattggccactctttcttggaaagtagtgttatatggaggttctagatcttccactgtgggtggttcttggacatgtagcgttatctctgtttcatcagtgcctgctatgttagtagcaacacatgtatatatgccagcatctgagggcgtggcttggtcgatgcttaaagttccgtctggattgctaacatggtgctctccatcaaccagcatagtgcttccacctttggaccaggtgattacaggaagaggagtcccttgagcattacatggaatatccactctttgaccaacttggactttgagatgtttaggtccacgctgtatctttggaggaacatggacatttaatttgacagcctgagtcacattcccagcaatatttgtggcaacacaaagatacatcccactatctgaagtgcgggtttcagtgatcttcattgaaccagaagggaggaatgtgtgtcttggagagaacggtgagatgagctgggtttctttggcccaagtaattatgggtggaggtaagctcttcacttcacatggaagtgttacctcttcccctgcaaggacggagatctcaacaggcttatcctgggacagtcctcgttgatctccaaacactctgggccttacatagactgttagctgcactttccttttggcgtagccggctgtattggtggcagtgcagacatactccccactctcctctcctccaggtgataccacatacagactaccatcagctcctgctgaaaacttagcactgctggttgaaatcagctctcctttcttggaccagatgacagacggtttgggatttccacttgctttgcatggtaaagttactggaatgccttcaattgtactgagtatctgctgcccatgctgaatggttggcagaacatgcacaaccacagaggtagttttgttattggtcccagcaacgttactggccacacaagtatattcaccaccatcctgaagctgaactctttcaatatggaggctcccatcactgcgcacagtgatgtaaggattttggagcaacatagctgaattcttaatccaccgacgttctggaatgggatttccagctaacagagtacagggcaaagtaagctgctgtccttcaataacattggccactgaagggctgattccaataagtggagcaacaagtccggtcactgttactgttgtctctgactggatctttccaaactggttttcagcttcacaaatataggttcctttatcacttgcccataagtttaaaataaagagagctcctgttcttagttggctgatggaactaactgaaaaaggtcttgagaaaattggcatgttgtctaatcttcgccatttgattgttggttctggataaccctgaacataacaaggtaatgtcacatttgagccaatttccatagacacatcagcaggttcttgtatgaaaactggaggtgagccaacatccagagttatcttgccagttgctcttccagcctcattgatggctacacaggtataatcgccagcatccagatcttgtgtttcttgaatcttcaaaagtcccaagagagggtcaataatgaggaatgttgagggcctcaactcaagatctcctttgaaccatttaacttgaggtggaggaataccagaggttttgcattccataacggttatatccccaagggcaaccaagagctcactctgaactaccatcaacttaggggcttcaatgtatctgagagtagaattctgtttatctgttccagctgaattacttgctaggcaaccatagatccctgcatctttgggagctgcatttttgataaataaggtaccatctgaggtcatcctatacctgtgtgaacccacgataaacatatcgttaacggtccaggcaatctttggtttgggataacctgttgcagaacacatgatggagacctcagaccctcctgtgaaagactgattcttgggcatcacagtgactttgggtggttcttgcactgtgaggaaaactgaagcggctgatgatccaccttcactagaaaccatacaatgatactctccagcatcgttgaatttcacactctttagctccaatgacagattagccaaggtcctaattctcgctggctctgccagtctgacatctctgtcattcctctgccaggttagattgtaatccaccgcactgatgatgagacatgttaaaactgctctctctccaggagtgactgtaacattgttaggcacttggatgaccggagggggctctgatacgtcaaaaaatgtctgtgcccgtccagtacctgcactgctgacagcaatgcattcatagaaaccttcgtcagacaaagtgacctttgcaatatctaagttcacactggcagattctttcaaatactggtctactccaagtgtaactccatttctgacaaagctcaaggtaaagggcaaaagactgtcaacagagcagggaatttggcccggctgcagatagtatcctggggttttctcaggcatcgtaactttgggagcatctgggacaatactagaaaaggaaacacttgatactctctggaagaggtaatcatctttatcatagcctgttactttgagaaagaaagcttcatttggtggtacaaagtcagaaatattccatatgccataaggttttcgatgtgggtaatatttaacaggaatagtcttaagagaacttcctgagatactcaaaagttcaagaagatctattctagctggagtggaaattccagaagtattgagcagtacataggtaggtattccttgcactggtctgctgactgtttttttgaagtccagggtgggctttcgagaaaagccagctcggaaatcaatagtactgaggccagtaatgcgaacagagtgccttccactgcttgaggtcttcactgtccacattccagcctctggctctttcacattcactactttggcagagttatggatatttaatagctcatgcaggccaaatcccttttttatcagcttccctaaaggattgcgaatttcaatcattggagaaggcccactcaaagacacagtgacctctttcaggctgggatcaaaaggaattctccaagtatttacagcctgttccaaatgatctgtggataaaaggtgaactttggaggcctgtactgcttcttctacccattttaatacctcattaacttgttttttgtccagatggaacacttgaccagaacttgtagaggcaatttcttcatagactttatatccaatatgggtcctgtcatcacaatctccagtcagaacaaatacgacttgtgactgtttctgttggataagttgcagcacctcatgggtgagccggtaatctttggaccgagcatcagtgaaaacatagatgaaagaaccaggaagagaaatttccaaggcaatttttatagctccaatactcatttctgggcaatcaccaccaccctgaacatacagttctctgagttcatattgaaatttcttgggatctgtggtaattgtcactgggccaatttctggatcatggaaaggcaccaacgcaaagttgaaaagaggtcttttaggtcttttcaaagacgtctccaaaattttggaagccccttcaatcacctgaactaaatcatcatacatagaaccagtcacatcaaacacaaaagccaacgtggaggccccctcgggaatttcctcagctctgatctctgactgggggctcgcatcttgagctagggaagaataaagaagagcaaacaggaatactgtatggacaacttcccaggaaatcattttcttttttttccccctctttttccccctcagcgcctaagcactgtgctcagtcctcctcaacaacaggcagagggtttcctctcagagtaactcatcagactcttggaatctctgaactagcaaaaagtttggcgctgagaatcagacggggacaagcaccaaactcgaatccctccaggggttgggcagggcagggatgcggcagcttttgtctggatgcggcttcctcctggactgctatctg

SEQ ID NO: 9640 - RNA, 6329 nt, Homo sapiens
  source 1..6329: mol_type = other RNA
atcccaccactgccaccatgttattgctgccagaaattgatggggccacatgaacttgcagactgtaaaataactctgtagctccagctgagttgatggccacgcatttatatatgccagcatctgagatctgggcactttcaatatcaatgatctgtcctctgttcaagaaagtcatgctggtggaacctgagagtagacgattatctttgtaccatgtaataacaggcacaggatttccagctgccttacactccagctgtacagggttgctcaccaacacagtctcattcagcatttttccagcatcttccagactaggtggttcatgaacatgcagttgaatgtgctgttgtgtttctccagctgcgttggtagccacacatgtgtatctgccagcatcttccaacagggttttggcaatttgtagaactcgaccagaagactgtattttaaggtttccttgggcagtgttcacaggctggtcatcttttaaccatgtaatggaaggatttggaatcccattggctatgcactgcaaggcgacaggcttgtattttaccacaactctctcagaaaggcctgaggacttgattgttggaggaacatgaacagtcacttcaaattccttcttgtggtctccagcagtatttgctgccatgcaccgataaaggcctgtgtttgacacttgagcctgagcaataaccagtttgcgtccatttaataaaatcttgaatccatccctttcatcaattaactggccatccttcagccacatgatagttggtgggggagagcctgtcacatgacaatctagctccagtaagttattaaccatcacaatgaagtaagatgtttcatctcctccttctatagctggtggcaccaagacatcaacttcatatttgatttccttttctcctgccacactggtagccacgcatatgtactgtcctcgatcaatttcttgggcactcatgatttcgagtttcttcccaccagcttctatgcggatattgtcattagctttcacaggtacaccatctttcaaccaggtgagaatgggagaagggtttccagcagctttgcactccagtgtcagagaatgagcaataactacttgcttattcaaaggcgtggccaagttgccttcaatcattggaggaacatagacatccacatggaatgatttttcagcagttccagcaacattggctacatgacacgtatatgttgctgaatcagagacctgtgctcgaggaatatgaagatattgtcctttatcaatataaagtgcttgtgagctggacatgattggctgcccgtccttataccaagtaatggcaggcattggaagtccccgtgtttcacattccagtttaataaggctgttgatcaatactgatatgtctgtggtgacatttcctcctttaatactaggtggaatatagatagtcagttttatatccttggcttgtttgccagctgcattagacacagtacattggtagcgccccttgtcatttctccgtgcattctttaaatgtaagacttgtcctctgtctagaagttcaacattaggatcgcccaaaaataaaggcttgccatctttgaaccaatgaatatcaggaaagggagtgcctttgacctggcattcaagggcgacgtcacggttgaggacaactgagacttcatttgggaagttggtacctattatggtgggtggaactagcacatcaatgttaaagtacttctgagaagtgcctgcaatattaattgctttgcaggaatatcttcctgcatcctctggagtggctctgaagagcttcagtatcttcccattgttcacagtctgaatagtgctgctttcagtcacctggacattatctttataccacataatgatgggagatggagtgccttccacttcacagaagagattggtcagctgatttaacaacaccgacacatttgtaacttgttctttatctttaattactggaggaacatggactttgaggttatattttctttctgtggttccagcttcattgactgccacacagatgtactccccattgtcatagggtgtaacagaagcaataaccagcaatgtgccatcttccaagatagaaatgccaggctctctgcctgtcaactctctaccattgtgtaaccatttgatggttggtttaggggtaccttttgcaggacatggaaattcaatgcgttgattggccactctttcttggaaagtagtgttatatggaggttctagatcttccactgtgggtggttcttggacatgtagcgttatctctgtttcatcagtgcctgctatgttagtagcaacacatgtatatatgccagcatctgagggcgtggcttggtcgatgcttaaagttccgtctggattgctaacatggtgctctccatcaaccagcatagtgcttccacctttggaccaggtgattacaggaagaggagtcccttgagcattacatggaatatccactctttgaccaacttggactttgagatgtttaggtccacgctgtatctttggaggaacatggacatttaatttgacagcctgagtcacattcccagcaatatttgtggcaacacaaagatacatcccactatctgaagtgcgggtttcagtgatcttcattgaaccagaagggaggaatgtgtgtcttggagagaacggtgagatgagctgggtttctttggcccaagtaattatgggtggaggtaagctcttcacttcacatggaagtgttacctcttcccctgcaaggacggagatctcaacaggcttatcctgggacagtcctcgttgatctccaaacactctgggccttacatagactgttagctgcactttccttttggcgtagccggctgtattggtggcagtgcagacatactccccactctcctctcctccaggtgataccacatacagactaccatcagctcctgctgaaaacttagcactgctggttgaaatcagctctcctttcttggaccagatgacagacggtttgggatttccacttgctttgcatggtaaagttactggaatgccttcaattgtactgagtatctgctgcccatgctgaatggttggcagaacatgcacaaccacagaggtagttttgttattggtcccagcaacgttactggccacacaagtatattcaccaccatcctgaagctgaactctttcaatatggaggctcccatcactgcgcacagtgatgtaaggattttggagcaacatagctgaattcttaatccaccgacgttctggaatgggatttccagctaacagagtacagggcaaagtaagctgctgtccttcaataacattggccactgaagggctgattccaataagtggagcaacaagtccggtcactgttactgttgtctctgactggatctttccaaactggttttcagcttcacaaatataggttcctttatcacttgcccataagtttaaaataaagagagctcctgttcttagttggctgatggaactaactgaaaaaggtcttgagaaaattggcatgttgtctaatcttcgccatttgattgttggttctggataaccctgaacataacaaggtaatgtcacatttgagccaatttccatagacacatcagcaggttcttgtatgaaaactggaggtgagccaacatccagagttatcttgccagttgctcttccagcctcattgatggctacacaggtataatcgccagcatccagatcttgtgtttcttgaatcttcaaaagtcccaagagagggtcaataatgaggaatgttgagggcctcaactcaagatctcctttgaaccatttaacttgaggtggaggaataccagaggttttgcattccataacggttatatccccaagggcaaccaagagctcactctgaactaccatcaacttaggggcttcaatgtatctgagagtagaattctgtttatctgttccagctgaattacttgctaggcaaccatagatccctgcatctttgggagctgcatttttgataaataaggtaccatctgaggtcatcctatacctgtgtgaacccacgataaacatatcgttaacggtccaggcaatctttggtttgggataacctgttgcagaacacatgatggagacctcagaccctcctgtgaaagactgattcttgggcatcacagtgactttgggtggttcttgcactgtgaggaaaactgaagcggctgatgatccaccttcactagaaaccatacaatgatactctccagcatcgttgaatttcacactctttagctccaatgacagattagccaaggtcctaattctcgctggctctgccagtctgacatctctgtcattcctctgccaggttagattgtaatccaccgcactgatgatgagacatgttaaaactgctctctctccaggagtgactgtaacattgttaggcacttggatgaccggagggggctctgatacgtcaaaaaatgtctgtgcccgtccagtacctgcactgctgacagcaatgcattcatagaaaccttcgtcagacaaagtgacctttgcaatatctaagttcacactggcagattctttcaaatactggtctactccaagtgtaactccatttctgacaaagctcaaggtaaagggcaaaagactgtcaacagagcagggaatttggcccggctgcagatagtatcctggggttttctcaggcatcgtaactttgggagcatctgggacaatactagaaaaggaaacacttgatactctctggaagaggtaatcatctttatcatagcctgttactttgagaaagaaagcttcatttggtggtacaaagtcagaaatattccatatgccataaggttttcgatgtgggtaatatttaacaggaatagtcttaagagaacttcctgagatactcaaaagttcaagaagatctattctagctggagtggaaattccagaagtattgagcagtacataggtaggtattccttgcactggtctgctgactgtttttttgaagtccagggtgggctttcgagaaaagccagctcggaaatcaatagtactgaggccagtaatgcgaacagagtgccttccactgcttgaggtcttcactgtccacattccagcctctggctctttcacattcactactttggcagagttatggatatttaatagctcatgcaggccaaatcccttttttatcagcttccctaaaggattgcgaatttcaatcattggagaaggcccactcaaagacacagtgacctctttcaggctgggatcaaaaggaattctccaagtatttacagcctgttccaaatgatctgtggataaaaggtgaactttggaggcctgtactgcttcttctacccattttaatacctcattaacttgttttttgtccagatggaacacttgaccagaacttgtagaggcaatttcttcatagactttatatccaatatgggtcctgtcatcacaatctccagtcagaacaaatacgacttgtgactgtttctgttggataagttgcagcacctcatgggtgagccggtaatctttggaccgagcatcagtgaaaacatagatgaaagaaccaggaagagaaatttccaaggcaatttttatagctccaatactcatttctgggcaatcaccaccaccctgaacatacagttctctgagttcatattgaaatttcttgggatctgtggtaattgtcactgggccaatttctggatcatggaaaggcaccaacgcaaagttgaaaagaggtcttttaggtcttttcaaagacgtctccaaaattttggaagccccttcaatcacctgaactaaatcatcatacatagaaccagtcacatcaaacacaaaagccaacgtggaggccccctcgggaatttcctcagctctgatctctgactgggggctcgcatcttgagctagggaagaataaagaagagcaaacaggaatactgtatggacaacttcccaggaaatcattttcttttttttccccctctttttccccctcagcgcctaagcactgtgctcagtcctcctcaacaacaggcagagggtttcctctcagagtaactcatcagactcttggaatctctgaactagcaaaaagtttggcgctgagaatcagacggggacaagcaccaaactcgaatccctccaggggttgggcagggcagggatgcggcagcttttgtctggatgcggcttcctcctggactgctatctgcccgcg

SEQ ID NO: 9641 - RNA, 6331 nt, Homo sapiens
  source 1..6331: mol_type = other RNA
atcccaccactgccaccatgttattgctgccagaaattgatggggccacatgaacttgcagactgtaaaataactctgtagctccagctgagttgatggccacgcatttatatatgccagcatctgagatctgggcactttcaatatcaatgatctgtcctctgttcaagaaagtcatgctggtggaacctgagagtagacgattatctttgtaccatgtaataacaggcacaggatttccagctgccttacactccagctgtacagggttgctcaccaacacagtctcattcagcatttttccagcatcttccagactaggtggttcatgaacatgcagttgaatgtgctgttgtgtttctccagctgcgttggtagccacacatgtgtatctgccagcatcttccaacagggttttggcaatttgtagaactcgaccagaagactgtattttaaggtttccttgggcagtgttcacaggctggtcatcttttaaccatgtaatggaaggatttggaatcccattggctatgcactgcaaggcgacaggcttgtattttaccacaactctctcagaaaggcctgaggacttgattgttggaggaacatgaacagtcacttcaaattccttcttgtggtctccagcagtatttgctgccatgcaccgataaaggcctgtgtttgacacttgagcctgagcaataaccagtttgcgtccatttaataaaatcttgaatccatccctttcatcaattaactggccatccttcagccacatgatagttggtgggggagagcctgtcacatgacaatctagctccagtaagttattaaccatcacaatgaagtaagatgtttcatctcctccttctatagctggtggcaccaagacatcaacttcatatttgatttccttttctcctgccacactggtagccacgcatatgtactgtcctcgatcaatttcttgggcactcatgatttcgagtttcttcccaccagcttctatgcggatattgtcattagctttcacaggtacaccatctttcaaccaggtgagaatgggagaagggtttccagcagctttgcactccagtgtcagagaatgagcaataactacttgcttattcaaaggcgtggccaagttgccttcaatcattggaggaacatagacatccacatggaatgatttttcagcagttccagcaacattggctacatgacacgtatatgttgctgaatcagagacctgtgctcgaggaatatgaagatattgtcctttatcaatataaagtgcttgtgagctggacatgattggctgcccgtccttataccaagtaatggcaggcattggaagtccccgtgtttcacattccagtttaataaggctgttgatcaatactgatatgtctgtggtgacatttcctcctttaatactaggtggaatatagatagtcagttttatatccttggcttgtttgccagctgcattagacacagtacattggtagcgccccttgtcatttctccgtgcattctttaaatgtaagacttgtcctctgtctagaagttcaacattaggatcgcccaaaaataaaggcttgccatctttgaaccaatgaatatcaggaaagggagtgcctttgacctggcattcaagggcgacgtcacggttgaggacaactgagacttcatttgggaagttggtacctattatggtgggtggaactagcacatcaatgttaaagtacttctgagaagtgcctgcaatattaattgctttgcaggaatatcttcctgcatcctctggagtggctctgaagagcttcagtatcttcccattgttcacagtctgaatagtgctgctttcagtcacctggacattatctttataccacataatgatgggagatggagtgccttccacttcacagaagagattggtcagctgatttaacaacaccgacacatttgtaacttgttctttatctttaattactggaggaacatggactttgaggttatattttctttctgtggttccagcttcattgactgccacacagatgtactccccattgtcatagggtgtaacagaagcaataaccagcaatgtgccatcttccaagatagaaatgccaggctctctgcctgtcaactctctaccattgtgtaaccatttgatggttggtttaggggtaccttttgcaggacatggaaattcaatgcgttgattggccactctttcttggaaagtagtgttatatggaggttctagatcttccactgtgggtggttcttggacatgtagcgttatctctgtttcatcagtgcctgctatgttagtagcaacacatgtatatatgccagcatctgagggcgtggcttggtcgatgcttaaagttccgtctggattgctaacatggtgctctccatcaaccagcatagtgcttccacctttggaccaggtgattacaggaagaggagtcccttgagcattacatggaatatccactctttgaccaacttggactttgagatgtttaggtccacgctgtatctttggaggaacatggacatttaatttgacagcctgagtcacattcccagcaatatttgtggcaacacaaagatacatcccactatctgaagtgcgggtttcagtgatcttcattgaaccagaagggaggaatgtgtgtcttggagagaacggtgagatgagctgggtttctttggcccaagtaattatgggtggaggtaagctcttcacttcacatggaagtgttacctcttcccctgcaaggacggagatctcaacaggcttatcctgggacagtcctcgttgatctccaaacactctgggccttacatagactgttagctgcactttccttttggcgtagccggctgtattggtggcagtgcagacatactccccactctcctctcctccaggtgataccacatacagactaccatcagctcctgctgaaaacttagcactgctggttgaaatcagctctcctttcttggaccagatgacagacggtttgggatttccacttgctttgcatggtaaagttactggaatgccttcaattgtactgagtatctgctgcccatgctgaatggttggcagaacatgcacaaccacagaggtagttttgttattggtcccagcaacgttactggccacacaagtatattcaccaccatcctgaagctgaactctttcaatatggaggctcccatcactgcgcacagtgatgtaaggattttggagcaacatagctgaattcttaatccaccgacgttctggaatgggatttccagctaacagagtacagggcaaagtaagctgctgtccttcaataacattggccactgaagggctgattccaataagtggagcaacaagtccggtcactgttactgttgtctctgactggatctttccaaactggttttcagcttcacaaatataggttcctttatcacttgcccataagtttaaaataaagagagctcctgttcttagttggctgatggaactaactgaaaaaggtcttgagaaaattggcatgttgtctaatcttcgccatttgattgttggttctggataaccctgaacataacaaggtaatgtcacatttgagccaatttccatagacacatcagcaggttcttgtatgaaaactggaggtgagccaacatccagagttatcttgccagttgctcttccagcctcattgatggctacacaggtataatcgccagcatccagatcttgtgtttcttgaatcttcaaaagtcccaagagagggtcaataatgaggaatgttgagggcctcaactcaagatctcctttgaaccatttaacttgaggtggaggaataccagaggttttgcattccataacggttatatccccaagggcaaccaagagctcactctgaactaccatcaacttaggggcttcaatgtatctgagagtagaattctgtttatctgttccagctgaattacttgctaggcaaccatagatccctgcatctttgggagctgcatttttgataaataaggtaccatctgaggtcatcctatacctgtgtgaacccacgataaacatatcgttaacggtccaggcaatctttggtttgggataacctgttgcagaacacatgatggagacctcagaccctcctgtgaaagactgattcttgggcatcacagtgactttgggtggttcttgcactgtgaggaaaactgaagcggctgatgatccaccttcactagaaaccatacaatgatactctccagcatcgttgaatttcacactctttagctccaatgacagattagccaaggtcctaattctcgctggctctgccagtctgacatctctgtcattcctctgccaggttagattgtaatccaccgcactgatgatgagacatgttaaaactgctctctctccaggagtgactgtaacattgttaggcacttggatgaccggagggggctctgatacgtcaaaaaatgtctgtgcccgtccagtacctgcactgctgacagcaatgcattcatagaaaccttcgtcagacaaagtgacctttgcaatatctaagttcacactggcagattctttcaaatactggtctactccaagtgtaactccatttctgacaaagctcaaggtaaagggcaaaagactgtcaacagagcagggaatttggcccggctgcagatagtatcctggggttttctcaggcatcgtaactttgggagcatctgggacaatactagaaaaggaaacacttgatactctctggaagaggtaatcatctttatcatagcctgttactttgagaaagaaagcttcatttggtggtacaaagtcagaaatattccatatgccataaggttttcgatgtgggtaatatttaacaggaatagtcttaagagaacttcctgagatactcaaaagttcaagaagatctattctagctggagtggaaattccagaagtattgagcagtacataggtaggtattccttgcactggtctgctgactgtttttttgaagtccagggtgggctttcgagaaaagccagctcggaaatcaatagtactgaggccagtaatgcgaacagagtgccttccactgcttgaggtcttcactgtccacattccagcctctggctctttcacattcactactttggcagagttatggatatttaatagctcatgcaggccaaatcccttttttatcagcttccctaaaggattgcgaatttcaatcattggagaaggcccactcaaagacacagtgacctctttcaggctgggatcaaaaggaattctccaagtatttacagcctgttccaaatgatctgtggataaaaggtgaactttggaggcctgtactgcttcttctacccattttaatacctcattaacttgttttttgtccagatggaacacttgaccagaacttgtagaggcaatttcttcatagactttatatccaatatgggtcctgtcatcacaatctccagtcagaacaaatacgacttgtgactgtttctgttggataagttgcagcacctcatgggtgagccggtaatctttggaccgagcatcagtgaaaacatagatgaaagaaccaggaagagaaatttccaaggcaatttttatagctccaatactcatttctgggcaatcaccaccaccctgaacatacagttctctgagttcatattgaaatttcttgggatctgtggtaattgtcactgggccaatttctggatcatggaaaggcaccaacgcaaagttgaaaagaggtcttttaggtcttttcaaagacgtctccaaaattttggaagccccttcaatcacctgaactaaatcatcatacatagaaccagtcacatcaaacacaaaagccaacgtggaggccccctcgggaatttcctcagctctgatctctgactgggggctcgcatcttgagctagggaagaataaagaagagcaaacaggaatactgtatggacaacttcccaggaaatcattttcttttttttccccctctttttccccctcagcgcctaagcactgtgctcagtcctcctcaacaacaggcagagggtttcctctcagagtaactcatcagactcttggaatctctgaactagcaaaaagtttggcgctgagaatcagacggggacaagcaccaaactcgaatccctccaggggttgggcagggcagggatgcggcagcttttgtctggatgcggcttcctcctggactgctatctgcccgcggg

SEQ ID NO: 9642 - RNA, 6465 nt, Homo sapiens
  source 1..6465: mol_type = other RNA
atcccaccactgccaccatgttattgctgccagaaattgatggggccacatgaacttgcagactgtaaaataactctgtagctccagctgagttgatggccacgcatttatatatgccagcatctgagatctgggcactttcaatatcaatgatctgtcctctgttcaagaaagtcatgctggtggaacctgagagtagacgattatctttgtaccatgtaataacaggcacaggatttccagctgccttacactccagctgtacagggttgctcaccaacacagtctcattcagcatttttccagcatcttccagactaggtggttcatgaacatgcagttgaatgtgctgttgtgtttctccagctgcgttggtagccacacatgtgtatctgccagcatcttccaacagggttttggcaatttgtagaactcgaccagaagactgtattttaaggtttccttgggcagtgttcacaggctggtcatcttttaaccatgtaatggaaggatttggaatcccattggctatgcactgcaaggcgacaggcttgtattttaccacaactctctcagaaaggcctgaggacttgattgttggaggaacatgaacagtcacttcaaattccttcttgtggtctccagcagtatttgctgccatgcaccgataaaggcctgtgtttgacacttgagcctgagcaataaccagtttgcgtccatttaataaaatcttgaatccatccctttcatcaattaactggccatccttcagccacatgatagttggtgggggagagcctgtcacatgacaatctagctccagtaagttattaaccatcacaatgaagtaagatgtttcatctcctccttctatagctggtggcaccaagacatcaacttcatatttgatttccttttctcctgccacactggtagccacgcatatgtactgtcctcgatcaatttcttgggcactcatgatttcgagtttcttcccaccagcttctatgcggatattgtcattagctttcacaggtacaccatctttcaaccaggtgagaatgggagaagggtttccagcagctttgcactccagtgtcagagaatgagcaataactacttgcttattcaaaggcgtggccaagttgccttcaatcattggaggaacatagacatccacatggaatgatttttcagcagttccagcaacattggctacatgacacgtatatgttgctgaatcagagacctgtgctcgaggaatatgaagatattgtcctttatcaatataaagtgcttgtgagctggacatgattggctgcccgtccttataccaagtaatggcaggcattggaagtccccgtgtttcacattccagtttaataaggctgttgatcaatactgatatgtctgtggtgacatttcctcctttaatactaggtggaatatagatagtcagttttatatccttggcttgtttgccagctgcattagacacagtacattggtagcgccccttgtcatttctccgtgcattctttaaatgtaagacttgtcctctgtctagaagttcaacattaggatcgcccaaaaataaaggcttgccatctttgaaccaatgaatatcaggaaagggagtgcctttgacctggcattcaagggcgacgtcacggttgaggacaactgagacttcatttgggaagttggtacctattatggtgggtggaactagcacatcaatgttaaagtacttctgagaagtgcctgcaatattaattgctttgcaggaatatcttcctgcatcctctggagtggctctgaagagcttcagtatcttcccattgttcacagtctgaatagtgctgctttcagtcacctggacattatctttataccacataatgatgggagatggagtgccttccacttcacagaagagattggtcagctgatttaacaacaccgacacatttgtaacttgttctttatctttaattactggaggaacatggactttgaggttatattttctttctgtggttccagcttcattgactgccacacagatgtactccccattgtcatagggtgtaacagaagcaataaccagcaatgtgccatcttccaagatagaaatgccaggctctctgcctgtcaactctctaccattgtgtaaccatttgatggttggtttaggggtaccttttgcaggacatggaaattcaatgcgttgattggccactctttcttggaaagtagtgttatatggaggttctagatcttccactgtgggtggttcttggacatgtagcgttatctctgtttcatcagtgcctgctatgttagtagcaacacatgtatatatgccagcatctgagggcgtggcttggtcgatgcttaaagttccgtctggattgctaacatggtgctctccatcaaccagcatagtgcttccacctttggaccaggtgattacaggaagaggagtcccttgagcattacatggaatatccactctttgaccaacttggactttgagatgtttaggtccacgctgtatctttggaggaacatggacatttaatttgacagcctgagtcacattcccagcaatatttgtggcaacacaaagatacatcccactatctgaagtgcgggtttcagtgatcttcattgaaccagaagggaggaatgtgtgtcttggagagaacggtgagatgagctgggtttctttggcccaagtaattatgggtggaggtaagctcttcacttcacatggaagtgttacctcttcccctgcaaggacggagatctcaacaggcttatcctgggacagtcctcgttgatctccaaacactctgggccttacatagactgttagctgcactttccttttggcgtagccggctgtattggtggcagtgcagacatactccccactctcctctcctccaggtgataccacatacagactaccatcagctcctgctgaaaacttagcactgctggttgaaatcagctctcctttcttggaccagatgacagacggtttgggatttccacttgctttgcatggtaaagttactggaatgccttcaattgtactgagtatctgctgcccatgctgaatggttggcagaacatgcacaaccacagaggtagttttgttattggtcccagcaacgttactggccacacaagtatattcaccaccatcctgaagctgaactctttcaatatggaggctcccatcactgcgcacagtgatgtaaggattttggagcaacatagctgaattcttaatccaccgacgttctggaatgggatttccagctaacagagtacagggcaaagtaagctgctgtccttcaataacattggccactgaagggctgattccaataagtggagcaacaagtccggtcactgttactgttgtctctgactggatctttccaaactggttttcagcttcacaaatataggttcctttatcacttgcccataagtttaaaataaagagagctcctgttcttagttggctgatggaactaactgaaaaaggtcttgagaaaattggcatgttgtctaatcttcgccatttgattgttggttctggataaccctgaacataacaaggtaatgtcacatttgagccaatttccatagacacatcagcaggttcttgtatgaaaactggaggtgagccaacatccagagttatcttgccagttgctcttccagcctcattgatggctacacaggtataatcgccagcatccagatcttgtgtttcttgaatcttcaaaagtcccaagagagggtcaataatgaggaatgttgagggcctcaactcaagatctcctttgaaccatttaacttgaggtggaggaataccagaggttttgcattccataacggttatatccccaagggcaaccaagagctcactctgaactaccatcaacttaggggcttcaatgtatctgagagtagaattctgtttatctgttccagctgaattacttgctaggcaaccatagatccctgcatctttgggagctgcatttttgataaataaggtaccatctgaggtcatcctatacctgtgtgaacccacgataaacatatcgttaacggtccaggcaatctttggtttgggataacctgttgcagaacacatgatggagacctcagaccctcctgtgaaagactgattcttgggcatcacagtgactttgggtggttcttgcactgtgaggaaaactgaagcggctgatgatccaccttcactagaaaccatacaatgatactctccagcatcgttgaatttcacactctttagctccaatgacagattagccaaggtcctaattctcgctggctctgccagtctgacatctctgtcattcctctgccaggttagattgtaatccaccgcactgatgatgagacatgttaaaactgctctctctccaggagtgactgtaacattgttaggcacttggatgaccggagggggctctgatacgtcaaaaaatgtctgtgcccgtccagtacctgcactgctgacagcaatgcattcatagaaaccttcgtcagacaaagtgacctttgcaatatctaagttcacactggcagattctttcaaatactggtctactccaagtgtaactccatttctgacaaagctcaaggtaaagggcaaaagactgtcaacagagcagggaatttggcccggctgcagatagtatcctggggttttctcaggcatcgtaactttgggagcatctgggacaatactagaaaaggaaacacttgatactctctggaagaggtaatcatctttatcatagcctgttactttgagaaagaaagcttcatttggtggtacaaagtcagaaatattccatatgccataaggttttcgatgtgggtaatatttaacaggaatagtcttaagagaacttcctgagatactcaaaagttcaagaagatctattctagctggagtggaaattccagaagtattgagcagtacataggtaggtattccttgcactggtctgctgactgtttttttgaagtccagggtgggctttcgagaaaagccagctcggaaatcaatagtactgaggccagtaatgcgaacagagtgccttccactgcttgaggtcttcactgtccacattccagcctctggctctttcacattcactactttggcagagttatggatatttaatagctcatgcaggccaaatcccttttttatcagcttccctaaaggattgcgaatttcaatcattggagaaggcccactcaaagacacagtgacctctttcaggctgggatcaaaaggaattctccaagtatttacagcctgttccaaatgatctgtggataaaaggtgaactttggaggcctgtactgcttcttctacccattttaatacctcattaacttgttttttgtccagatggaacacttgaccagaacttgtagaggcaatttcttcatagactttatatccaatatgggtcctgtcatcacaatctccagtcagaacaaatacgacttgtgactgtttctgttggataagttgcagcacctcatgggtgagccggtaatctttggaccgagcatcagtgaaaacatagatgaaagaaccaggaagagaaatttccaaggcaatttttatagctccaatactcatttctgggcaatcaccaccaccctgaacatacagttctctgagttcatattgaaatttcttgggatctgtggtaattgtcactgggccaatttctggatcatggaaaggcaccaacgcaaagttgaaaagaggtcttttaggtcttttcaaagacgtctccaaaattttggaagccccttcaatcacctgaactaaatcatcatacatagaaccagtcacatcaaacacaaaagccaacgtggaggccccctcgggaatttcctcagctctgatctctgactgggggctcgcatcttgagctagggaagaataaagaagagcaaacaggaatactgtatggacaacttcccaggaaatcattttcttttttttccccctctttttccccctcagcgcctaagcactgtgctcagtcctcctcaacaacaggcagagggtttcctctcagagtaactcatcagactcttggaatctctgaactagcaaaaagtttggcgctgagaatcagacggggacaagcaccaaactcgaatccctccaggggttgggcagggcagggatgcggcagcttttgtctggatgcggcttcctcctggactgctatctgcccgcgggccctggacagcctgtggcggagtgcgggcggcgcgtcgggtccatgccccgggggcagctctgagcctgcggcgccgcggcccgaatcccgctgccctcgccgccgccgctgctctccgcctgggccagcgact

SEQ ID NO: 9643 - RNA, 1749 nt, Homo sapiens
  source 1..1749: mol_type = other RNA
atcccaccactgccaccattattgctactgttcagcaggtgctgctggtggtgatggtgatagtctggtgggggcggtggggctgctgttgctgctgcttgggaggccgcaggaggggcagcagggggcggtggaggggctgtagtggtggcagcagtggcggtggccttggtgtgtttgccagctttccttgccccctggccatgctgtacaaggctcaggagctgcaaggtgctttctctttcccggtctgagctctcggccctacctcgttcatatcgtccttcacagctcaggtggtgttggcggcagacagcgatccgagcccggaggcgctccacgatagcactgtgcactctcggggtgactgagccccctccaaggagccccgccccagaggccccccctagccctcctgcgggggcctgcgggggcgctgtgtcccccatcttaccggacacaatgattgctgcctctgggatggtgaggtggaaagaggctactgctggctattgcaggcaagtctgtttttgacaatgtgagctcagtgttcagggccacatgaatagaggtcttcagaggttgtgggggagccgtggagaagttgtgggggaggggagttagtaaaaagagggtggggagaaagaatagaaaccaactggggggaggataagttggaaacaaaccctgattaacttactctaattgcatttgacagctctggagaagttggacagagttggtggattttttttcctccaccaagctgacaagagccactaggtactttgtaaacacacgatctgggggttagatcaagaattcagggattgtccagcaagagacagaaacacacagcaaaaggtattgagagaggtattaatagagaggactccccctcacctagttgtttccgacaattctttatggggatgtttctgcagagaaacacatttctaccatgtctatgtaaccagcagccttgacttttcctcaggttaaataaaaaaccaaaacaaaacaaaacagtgctgtttcagaagatgtttaagtcactgttcaaaatgtgcaaaaatcaagggagactgtcttttggcttttaatttttcctccctttcctttcgctccggtgttttctcctctttggggtactgtaggatgttgtcttctcccaaaagagggagacagcttttcaactgttaacaatgtcagtaattggacttttggaccatgcttttttcttcagctaatccaatcaccggtaaaatcctcactccctctaaggtttcctagccttaaatgaaaagcaatcttaagtcgctagccactgagagagatccttcaacacatttttttctttcccgcttacgtttctattcctcacccccggctctattctaatacagtatcaagagagacaaactcttccgagagtaatttacaaacgatggtcaaacttacaaacttccagcaaattgcaccgagtcatgtccagccacttttctgtccacttttgtacattccatccccggccagtggatctgagggtctggactcgcaataagcaatctggttctatctcctgtatttgctccgctttatagatggaaaaaaaaagtagcttgtattttcctttctctttctcgtctgttgttagccgctttgctgacactggctcgcgcccggagtcacggcgatacacaggctttcattgtgctccgataggagagggagagaaagagagagagt

SEQ ID NO: 9644 - RNA, 1862 nt, Homo sapiens
  source 1..1862: mol_type = other RNA
atcccaccactgccaccattattgctactgttcagcaggtgctgctggtggtgatggtgatagtctggtgggggcggtggggctgctgttgctgctgcttgggaggccgcaggaggggcagcagggggcggtggaggggctgtagtggtggcagcagtggcggtggccttggtgtgtttgccagctttccttgccccctggccatgctgtacaaggctcaggagctgcaaggtgctttctctttcccggtctgagctctcggccctacctcgttcatatcgtccttcacagctcaggtggtgttggcggcagacagcgatccgagcccggaggcgctccacgatagcactgtgcactctcggggtgactgagccccctccaaggagccccgccccagaggccccccctagccctcctgcgggggcctgcgggggcgctgtgtcccccatcttaccggacacaatgattgctgcctctgggatggtgaggtggaaagaggctactgctggctattgcaggcaagtctgtttttgacaatgtgagctcagtgttcagggccacatgaatagaggtcttcagaggttgtgggggagccgtggagaagttgtgggggaggggagttagtaaaaagagggtggggagaaagaatagaaaccaactggggggaggataagttggaaacaaaccctgattaacttactctaattgcatttgacagctctggagaagttggacagagttggtggattttttttcctccaccaagctgacaagagccactaggtactttgtaaacacacgatctgggggttagatcaagaattcagggattgtccagcaagagacagaaacacacagcaaaaggtattgagagaggtattaatagagaggactccccctcacctagttgtttccgacaattctttatggggatgtttctgcagagaaacacatttctaccatgtctatgtaaccagcagccttgacttttcctcaggttaaataaaaaaccaaaacaaaacaaaacagtgctgtttcagaagatgtttaagtcactgttcaaaatgtgcaaaaatcaagggagactgtcttttggcttttaatttttcctccctttcctttcgctccggtgttttctcctctttggggtactgtaggatgttgtcttctcccaaaagagggagacagcttttcaactgttaacaatgtcagtaattggacttttggaccatgcttttttcttcagctaatccaatcaccggtaaaatcctcactccctctaaggtttcctagccttaaatgaaaagcaatcttaagtcgctagccactgagagagatccttcaacacatttttttctttcccgcttacgtttctattcctcacccccggctctattctaatacagtatcaagagagacaaactcttccgagagtaatttacaaacgatggtcaaacttacaaacttccagcaaattgcaccgagtcatgtccagccacttttctgtccacttttgtacattccatccccggccagtggatctgagggtctggactcgcaataagcaatctggttctatctcctgtatttgctccgctttatagatggaaaaaaaaagtagcttgtattttcctttctctttctcgtctgttgttagccgctttgctgacactggctcgcgcccggagtcacggcgatacacaggctttcattgtgctccgataggagagggagagaaagagagagagtgagacagagaaggagaaagagagagccagcaagctgcagatgggggtgggggggcggggagagggcgggagagctcgttcgaggctccctggtggaaggctggtgccactgcg

SEQ ID NO: 9645 - RNA, 1030 nt, Homo sapiens
  source 1..1030: mol_type = other RNA
atcccacctctgccaccaaaacactcatcgcggggtcagagggagtgccaaaaaaggtaaaaagaaacgcaagaaagaggctactggggatgaggggacacccagaagccccttcctggaggaaaagccactccttctgcagctggactctaggatactgagacccagccctgccccatcacctctccagtgtggccaaggggacaaggaccaagatgcagggaagcttggggagcctgggctacaacagatacaggccaacagacagacacagatggatgggggctgccgggcggggtcgcctcttactcgccatcccagcctcgactcatggcctgcactacggccccgtagagttggctccaggcagcccgtgtggctggtgtgaaggcagggcccagacacttctccagcatgtagagcagagactcacccactgtcgagaaggagctgagcttcacacccactgcccggtgcttcctgcccaggctggcaaggtactcctccagtgaggacaggtcttccacattggtcactgcagcatcaatcacgagcatcaccttcctgatgtggtccaggaactcaggcgaggagagacagtcctctgggctggagaactggcggcagttgtactggaagaggggcagcaggtcaggctccagggcaaacagcctggcaaacaggacggtgccgtgctccagcgggctgcggctcactgcccgccagctctgccggatcagctcgggctccgggcgctccatgctgtcccggggacgcggagcgcggggctgggaccctcagggctcgggtgccgtcaccgcacgtgccgcgccatctcctccgcgacgcggtcccctccgcccctcgtacgccccccgtgcctccgcccggcgggggccgcagccgctccttccctggcgcgggagagaaaaggcgcgcggccagtcgtaggtggagacaccccagctgtgcttccggggaccccgcttggccgctgcgccctgcgccccgcagccgccagagccgcccc

SEQ ID NO: 9646 - RNA, 317 nt, Homo sapiens
  source 1..317: mol_type = other RNA
atcccacctctgccaccaagagatcatcgctggaagccgagttttcagcaagacgcttgaactcatcctgcttctcaccgtaggggtactgggtgtcgaacttcaccaagacgaacttgcttttgggaatgaccttgtagaaagtgaccgtatccaggggaagggcgcccttggtgtgcaggccgctgccgccatgcggagcggagaggagcaggaagcccaggagaaggggaagcagcggggagagaaatgcggcgcggggcacagcggcagccatatcgccgggttcctgcagagggaggtaggtaagcgatagt

SEQ ID NO: 9647 - RNA, 1073 nt, Homo sapiens
  source 1..1073: mol_type = other RNA
atcccacctctgccaccaccacgccctctgccaccacggaaaccaagacctcctctgcctctgtatcccccacggccacggtttggacgaagtgggattccaaatgtttcagcatttaatcttctttcttcagcccaggttggtctccgttctctacttgtctcttgttatcatttctgagttgctcattttctggccttgaaactttgtgtacttcagctcgcctgtgctcctgattctctcctgccttttggctggcagatggcaaaggcctggttgatacaggactccttctcccaacagctgctggagcaggtaagtgggctgaggcggtctgcactgcttgttccatggttgggctttttctcaaagggtctaactgagggcttgagcgaccttgagataactgtgtttttagagatcttgtatcctgtgtaaaggcagaaccaaccgcactactttggggtaaggtaccactgtttgatgtttctgttccaaaggatgtcaaagagcttccagcaacaccaacagcaccaaactgctgcccaactaaggaactcggactgaactgactgtatgtgggcatcctgccgaaaggtccataagaacccatggactggaatgaagaagtcgatgagcctagtgaggactgaacaatagctgggtcttgaggcaaagaacactgtggttttggtggctcacaaacagtaaggtctttaatgtcactcccacggaatataatgtattcaaagacttcatctcgaggtggtattggacgatctgtcggtctgtcttctgtaccaaaggatcgaactttggcaagggctacggtggagttttcggtgtcgatggtgtagaggatgccctcgtagcggatctccgccttggagatgaggctgatcttgctgccgatgtaaggggtgcccccgctcatggcgccgccgccgccgctcccagctgctcgcagagaggcagatcccacgccactgtcgcccgctccgcacgcccgctcgctccgtcggcgcctacagcagccgcttcagacccaacatggcggcggcgccggctccgct

SEQ ID NO: 9648 - RNA, 1448 nt, Homo sapiens
  source 1..1448: mol_type = other RNA
atcccacctctgccaccaccacgccctctgccaccacggaaaccaagacctcctctgcctctgtatcccccacggccacggtttggacgaagtgggattccaaatgtttcagcatttaatcttctttcttcagcccaggttggtctccgttctctattataaaagcaaataatctattgtcatcacaagaaatattatcaaagaaggatttagttttgtcataatagcaattaggtccaagtggatcttcttcatcggcatttccttcactgttttgggtatcaactcctgagtctcctttatcttcaccatttacaggcttctcctgtttctcaagtttatcttcttttaatttaagtttattatgaaactctctgtcaatctcttccttgttgaattgtgcatttgcactttcaaagtcaaagtctttctcaaatttcattggcccatctcgccgaataccaaatcttcccctgccaccccgatgacccccacgccctctccttggagctgaaggagcacctggagctacttgtctcttgttatcatttctgagttgctcattttctggccttgaaactttgtgtacttcagctcgcctgtgctcctgattctctcctgccttttggctggcagatggcaaaggcctggttgatacaggactccttctcccaacagctgctggagcaggtaagtgggctgaggcggtctgcactgcttgttccatggttgggctttttctcaaagggtctaactgagggcttgagcgaccttgagataactgtgtttttagagatcttgtatcctgtgtaaaggcagaaccaaccgcactactttggggtaaggtaccactgtttgatgtttctgttccaaaggatgtcaaagagcttccagcaacaccaacagcaccaaactgctgcccaactaaggaactcggactgaactgactgtatgtgggcatcctgccgaaaggtccataagaacccatggactggaatgaagaagtcgatgagcctagtgaggactgaacaatagctgggtcttgaggcaaagaacactgtggttttggtggctcacaaacagtaaggtctttaatgtcactcccacggaatataatgtattcaaagacttcatctcgaggtggtattggacgatctgtcggtctgtcttctgtaccaaaggatcgaactttggcaagggctacggtggagttttcggtgtcgatggtgtagaggatgccctcgtagcggatctccgccttggagatgaggctgatcttgctgccgatgtaaggggtgcccccgctcatggcgccgccgccgccgctcccagctgctcgcagagaggcagatcccacgccactgtcgcccgctccgcacgcccgctcgctccgtcggcgcctacagcagccgcttcagacccaacatggcggcggcgccggctccgct

SEQ ID NO: 9649 - RNA, 1245 nt, Homo sapiens
  source 1..1245: mol_type = other RNA
atcccacctctgccaccaccacgccctctgccaccacggaaaccaagacctcctctgcctctgtatcccccacggccacggtttggacgaagtgggattccaaatgtttcagcatttaatcttctttcttcagcccaggttggtctccgttctctattgtcatcacaagaaatattatcaaagaaggatttagttttgtcataatagcaattaggtccaagtggatcttcttcatcggcatttccttcactgttttgggtatcaactcctgagtctcctttatcttcaccatttacaggcttctcctgtttctcaagtttatcttctacttgtctcttgttatcatttctgagttgctcattttctggccttgaaactttgtgtacttcagctcgcctgtgctcctgattctctcctgccttttggctggcagatggcaaaggcctggttgatacaggactccttctcccaacagctgctggagcaggtaagtgggctgaggcggtctgcactgcttgttccatggttgggctttttctcaaagggtctaactgagggcttgagcgaccttgagataactgtgtttttagagatcttgtatcctgtgtaaaggcagaaccaaccgcactactttggggtaaggtaccactgtttgatgtttctgttccaaaggatgtcaaagagcttccagcaacaccaacagcaccaaactgctgcccaactaaggaactcggactgaactgactgtatgtgggcatcctgccgaaaggtccataagaacccatggactggaatgaagaagtcgatgagcctagtgaggactgaacaatagctgggtcttgaggcaaagaacactgtggttttggtggctcacaaacagtaaggtctttaatgtcactcccacggaatataatgtattcaaagacttcatctcgaggtggtattggacgatctgtcggtctgtcttctgtaccaaaggatcgaactttggcaagggctacggtggagttttcggtgtcgatggtgtagaggatgccctcgtagcggatctccgccttggagatgaggctgatcttgctgccgatgtaaggggtgcccccgctcatggcgccgccgccgccgctcccagctgctcgcagagaggcagatcccacgccactgtcgcccgctccgcacgcccgctcgctccgtcggcgcctacagcagccgcttcagacccaacatggcggcggcgccggctccgct

SEQ ID NO: 9650 - RNA, 1250 nt, Homo sapiens
  source 1..1250: mol_type = other RNA
atcccacctctgccaccaccacgccctctgccaccacggaaaccaagacctcctctgcctctgtatcccccacggccacggtttggacgaagtgggattccaaatgtttcagcatttaatcttctttcttcagcccaggttggtctccgttctctattgtcatcacaagaaatattatcaaagaaggatttagttttgtcataatagcaattaggtccaagtggatcttcttcatcggcatttccttcactgttttgggtatcaactcctgagtctcctttatcttcaccatttacaggcttctcctgtttctcaagtttatcttctacttgtctcttgttatcatttctgagttgctcattttctggccttgaaactttgtgtacttcagctcgcctgtgctcctgattctctcctgccttttggctggcagatggcaaaggcctggttgatacaggactccttctcccaacagctgctggagcaggtaagtgggctgaggcggtctgcactgcttgttccatggttgggctttttctcaaagggtctaactgagggcttgagcgaccttgagataactgtgtttttagagatcttgtatcctgtgtaaaggcagaaccaaccgcactactttggggtaaggtaccactgtttgatgtttctgttccaaaggatgtcaaagagcttccagcaacaccaacagcaccaaactgctgcccaactaaggaactcggactgaactgactgtatgtgggcatcctgccgaaaggtccataagaacccatggactggaatgaagaagtcgatgagcctagtgaggactgaacaatagctgggtcttgaggcaaagaacactgtggttttggtggctcacaaacagtaaggtctttaatgtcactcccacggaatataatgtattcaaagacttcatctcgaggtggtattggacgatctgtcggtctgtcttctgtaccaaaggatcgaactttggcaagggctacggtggagttttcggtgtcgatggtgtagaggatgccctcgtagcggatctccgccttggagatgaggctgatcttgctgccgatgtaaggggtgcccccgctcatggcgccgccgccgccgctcccagctgctcgcagagaggcagatcccacgccactgtcgcccgctccgcacgcccgctcgctccgtcggcgcctacagcagccgcttcagacccaacatggcggcggcgccggctccgctaccct

SEQ ID NO: 9651 - RNA, 1299 nt, Homo sapiens
  source 1..1299: mol_type = other RNA
atcccacctctgccaccaccacgccctctgccaccacggaaaccaagacctcctctgcctctgtatcccccacggccacggtttggacgaagtgggattccaaatgtttcagcatttaatcttctttcttcagcccaggttggtctccgttctctattgtcatcacaagaaatattatcaaagaaggatttagttttgtcataatagcaattaggtccaagtggatcttcttcatcggcatttccttcactgttttgggtatcaactcctgagtctcctttatcttcaccatttacaggcttctcctgtttctcaagtttatcttctacttgtctcttgttatcatttctgagttgctcattttctggccttgaaactttgtgtacttcagctcgcctgtgctcctgattctctcctgccttttggctggcagatggcaaaggcctggttgatacaggactccttctcccaacagctgctggagcaggtaagtgggctgaggcggtctgcactgcttgttccatggttgggctttttctcaaagggtctaactgagggcttgagcgaccttgagataactgtgtttttagagatcttgtatcctgtgtaaaggcagaaccaaccgcactactttggggtaaggtaccactgtttgatgtttctgttccaaaggatgtcaaagagcttccagcaacaccaacagcaccaaactgctgcccaactaaggaactcggactgaactgactgtatgtgggcatcctgccgaaaggtccataagaacccatggactggaatgaagaagtcgatgagcctagtgaggactgggaggcggaggttgtagtgagccgagttcacgccactgtactccaacgactctgaacaatagctgggtcttgaggcaaagaacactgtggttttggtggctcacaaacagtaaggtctttaatgtcactcccacggaatataatgtattcaaagacttcatctcgaggtggtattggacgatctgtcggtctgtcttctgtaccaaaggatcgaactttggcaagggctacggtggagttttcggtgtcgatggtgtagaggatgccctcgtagcggatctccgccttggagatgaggctgatcttgctgccgatgtaaggggtgcccccgctcatggcgccgccgccgccgctcccagctgctcgcagagaggcagatcccacgccactgtcgcccgctccgcacgcccgctcgctccgtcggcgcctacagcagccgcttcagacccaacatggcggcggcgccggctccgct

SEQ ID NO: 9652 - RNA, 1068 nt, Homo sapiens
  source 1..1068: mol_type = other RNA
atcccacctctgccaccaccacgccctctgccaccacggaaaccaagacctcctctgcctctgtatcccccacggccacggtttggacgaagtgggattccaaatgtttcagcatttaatcttctttcttcagcccaggttggtctccgttctctattgtcatcacaagaaatattatcaaagaaggatttagttttgtcataatagcaattaggtccaagtggatcttcttcatcggcatttccttcactgttttgggtatcaactcctgagtctcctttatcttcaccatttacaggcttctcctgtttctcaagtttatcttctacttgtctcttgttatcatttctgagttgctcattttctggccttgaaactttgtgtacttcagcttgagataactgtgtttttagagatcttgtatcctgtgtaaaggcagaaccaaccgcactactttggggtaaggtaccactgtttgatgtttctgttccaaaggatgtcaaagagcttccagcaacaccaacagcaccaaactgctgcccaactaaggaactcggactgaactgactgtatgtgggcatcctgccgaaaggtccataagaacccatggactggaatgaagaagtcgatgagcctagtgaggactgaacaatagctgggtcttgaggcaaagaacactgtggttttggtggctcacaaacagtaaggtctttaatgtcactcccacggaatataatgtattcaaagacttcatctcgaggtggtattggacgatctgtcggtctgtcttctgtaccaaaggatcgaactttggcaagggctacggtggagttttcggtgtcgatggtgtagaggatgccctcgtagcggatctccgccttggagatgaggctgatcttgctgccgatgtaaggggtgcccccgctcatggcgccgccgccgccgctcccagctgctcgcagagaggcagatcccacgccactgtcgcccgctccgcacgcccgctcgctccgtcggcgcctacagcagccgcttcagacccaacatggcggcggcgccggctccgct

SEQ ID NO: 9653 - RNA, 1073 nt, Homo sapiens
  source 1..1073: mol_type = other RNA
atcccacctctgccaccaccacgccctctgccaccacggaaaccaagacctcctctgcctctgtatcccccacggccacggtttggacgaagtgggattccaaatgtttcagcatttaatcttctttcttcagcccaggttggtctccgttctctattgtcatcacaagaaatattatcaaagaaggatttagttttgtcataatagcaattaggtccaagtggatcttcttcatcggcatttccttcactgttttgggtatcaactcctgagtctcctttatcttcaccatttacaggcttctcctgtttctcaagtttatcttctacttgtctcttgttatcatttctgagttgctcattttctggccttgaaactttgtgtacttcagcttgagataactgtgtttttagagatcttgtatcctgtgtaaaggcagaaccaaccgcactactttggggtaaggtaccactgtttgatgtttctgttccaaaggatgtcaaagagcttccagcaacaccaacagcaccaaactgctgcccaactaaggaactcggactgaactgactgtatgtgggcatcctgccgaaaggtccataagaacccatggactggaatgaagaagtcgatgagcctagtgaggactgaacaatagctgggtcttgaggcaaagaacactgtggttttggtggctcacaaacagtaaggtctttaatgtcactcccacggaatataatgtattcaaagacttcatctcgaggtggtattggacgatctgtcggtctgtcttctgtaccaaaggatcgaactttggcaagggctacggtggagttttcggtgtcgatggtgtagaggatgccctcgtagcggatctccgccttggagatgaggctgatcttgctgccgatgtaaggggtgcccccgctcatggcgccgccgccgccgctcccagctgctcgcagagaggcagatcccacgccactgtcgcccgctccgcacgcccgctcgctccgtcggcgcctacagcagccgcttcagacccaacatggcggcggcgccggctccgctaccct

SEQ ID NO: 9654 - RNA, 1422 nt, Homo sapiens
  source 1..1422: mol_type = other RNA
atcccacctctgccaccaccacgccctctgccaccacggaaaccaagacctcctctgcctctgtatcccccacggccacggtttggacgaagtgggattccaaatgtttcagcatttaatcttctttcttcagcccaggttggtctccgttctctattgtcatcacaagaaatattatcaaagaaggatttagttttgtcataatagcaattaggtccaagtggatcttcttcatcggcatttccttcactgttttgggtatcaactcctgagtctcctttatcttcaccatttacaggcttctcctgtttctcaagtttatcttcttttaatttaagtttattatgaaactctctgtcaatctcttccttgttgaattgtgcatttgcactttcaaagtcaaagtctttctcaaatttcattggcccatctcgccgaataccaaatcttcccctgccaccccgatgacccccacgccctctccttggagctgaaggagcacctacttgtctcttgttatcatttctgagttgctcattttctggccttgaaactttgtgtacttcagctcgcctgtgctcctgattctctcctgccttttggctggcagatggcaaaggcctggttgatacaggactccttctcccaacagctgctggagcaggtaagtgggctgaggcggtctgcactgcttgttccatggttgggctttttctcaaagggtctaactgagggcttgagcgaccttgagataactgtgtttttagagatcttgtatcctgtgtaaaggcagaaccaaccgcactactttggggtaaggtaccactgtttgatgtttctgttccaaaggatgtcaaagagcttccagcaacaccaacagcaccaaactgctgcccaactaaggaactcggactgaactgactgtatgtgggcatcctgccgaaaggtccataagaacccatggactggaatgaagaagtcgatgagcctagtgaggactgaacaatagctgggtcttgaggcaaagaacactgtggttttggtggctcacaaacagtaaggtctttaatgtcactcccacggaatataatgtattcaaagacttcatctcgaggtggtattggacgatctgtcggtctgtcttctgtaccaaaggatcgaactttggcaagggctacggtggagttttcggtgtcgatggtgtagaggatgccctcgtagcggatctccgccttggagatgaggctgatcttgctgccgatgtaaggggtgcccccgctcatggcgccgccgccgccgctcccagctgctcgcagagaggcagatcccacgccactgtcgcccgctccgcacgcccgctcgctccgtcggcgcctacagcagccgcttcagacccaacatggcggcggcgccggctccgct

SEQ ID NO: 9655 - RNA, 1305 nt, Homo sapiens
  source 1..1305: mol_type = other RNA
atcccacctctgccaccaccacgccctctgccaccacggaaaccaagacctcctctgcctctgtatcccccacggccacggtttggacgaagtgggattccaaatgtttcagcatttaatcttctttcttcagcccaggttggtctccgttctctattgtcatcacaagaaatattatcaaagaaggatttagttttgtcataatagcaattaggtccaagtggatcttcttcatcggcatttccttcactgttttgggtatcaactcctgagtctcctttatcttcaccatttacaggcttctcctgtttctcaagtttatcttcttttaatttaagtttattatgaaactctctgtcaatctcttccttgttgaattgtgcatttgcactttcaaagtcaaagtctttctcaaatttcattggcccatctcgccgaataccaaatcttcccctgccaccccgatgacccccacgccctctccttggagctgaaggagcacctggagctacttgtctcttgttatcatttctgagttgctcattttctggccttgaaactttgtgtacttcagctcgcctgtgctcctgattctctcctgccttttggctggcagatggcaaaggcctggttgatacaggactccttctcccaacagctgctggagcaggtaagtgggctgaggcggtctgcactgcttgttccatggttgggctttttctcaaagggtctaactgagggcttgagcgaccaacaccaacagcaccaaactgctgcccaactaaggaactcggactgaactgactgtatgtgggcatcctgccgaaaggtccataagaacccatggactggaatgaagaagtcgatgagcctagtgaggactgaacaatagctgggtcttgaggcaaagaacactgtggttttggtggctcacaaacagtaaggtctttaatgtcactcccacggaatataatgtattcaaagacttcatctcgaggtggtattggacgatctgtcggtctgtcttctgtaccaaaggatcgaactttggcaagggctacggtggagttttcggtgtcgatggtgtagaggatgccctcgtagcggatctccgccttggagatgaggctgatcttgctgccgatgtaaggggtgcccccgctcatggcgccgccgccgccgctcccagctgctcgcagagaggcagatcccacgccactgtcgcccgctccgcacgcccgctcgctccgtcggcgcctacagcagccgcttcagacccaacatggcggcggcgccggctccgct

SEQ ID NO: 9656 - RNA, 1395 nt, Homo sapiens
  source 1..1395: mol_type = other RNA
atcccacctctgccaccaccacgccctctgccaccacggaaaccaagacctcctctgcctctgtatcccccacggccacggtttggacgaagtgggattccaaatgtttcagcatttaatcttctttcttcagcccaggttggtctccgttctctattgtcatcacaagaaatattatcaaagaaggatttagttttgtcataatagcaattaggtccaagtggatcttcttcatcggcatttccttcactgttttgggtatcaactcctgagtctcctttatcttcaccatttacaggcttctcctgtttctcaagtttatcttcttttaatttaagtttattatgaaactctctgtcaatctcttccttgttgaattgtgcatttgcactttcaaagtcaaagtctttctcaaatttcattggcccatctcgccgaataccaaatcttcccctgccaccccgatgacccccacgccctctccttggagctgaaggagcacctggagctacttgtctcttgttatcatttctgagttgctcattttctggccttgaaactttgtgtacttcagctcgcctgtgctcctgattctctcctgccttttggctggcagatggcaaaggcctggttgatacaggactccttctcccaacagctgctggagcaggtaagtgggctgaggcggtctgcactgcttgttccatggttgggctttttctcaaagggtctaactgagggcttgagcgaccttgagataactgtgtttttagagatcttgtatcctgtgtaaaggcagaaccaaccgcactactttggggtaaggtaccactgtttgatgtttctgttccaaaggatgtcaaagagcttccagcaacaccaacagcaccaaactgctgcccaactaaggaactcggactgaactgactgtatgtgggcatcctgccgaaaggtccataagaacccatggactgaacaatagctgggtcttgaggcaaagaacactgtggttttggtggctcacaaacagtaaggtctttaatgtcactcccacggaatataatgtattcaaagacttcatctcgaggtggtattggacgatctgtcggtctgtcttctgtaccaaaggatcgaactttggcaagggctacggtggagttttcggtgtcgatggtgtagaggatgccctcgtagcggatctccgccttggagatgaggctgatcttgctgccgatgtaaggggtgcccccgctcatggcgccgccgccgccgctcccagctgctcgcagagaggcagatcccacgccactgtcgcccgctccgcacgcccgctcgctccgtcggcgcctacagcagccgcttcagacccaacatggcggcggcgccggctccgct

SEQ ID NO: 9657 - RNA, 1438 nt, Homo sapiens
  source 1..1438: mol_type = other RNA
atcccacctctgccaccaccacgccctctgccaccacggaaaccaagacctcctctgcctctgtatcccccacggccacggtttggacgaagtgggattccaaatgtttcagcatttaatcttctttcttcagcccaggttggtctccgttctctattgtcatcacaagaaatattatcaaagaaggatttagttttgtcataatagcaattaggtccaagtggatcttcttcatcggcatttccttcactgttttgggtatcaactcctgagtctcctttatcttcaccatttacaggcttctcctgtttctcaagtttatcttcttttaatttaagtttattatgaaactctctgtcaatctcttccttgttgaattgtgcatttgcactttcaaagtcaaagtctttctcaaatttcattggcccatctcgccgaataccaaatcttcccctgccaccccgatgacccccacgccctctccttggagctgaaggagcacctggagctacttgtctcttgttatcatttctgagttgctcattttctggccttgaaactttgtgtacttcagctcgcctgtgctcctgattctctcctgccttttggctggcagatggcaaaggcctggttgatacaggactccttctcccaacagctgctggagcaggtaagtgggctgaggcggtctgcactgcttgttccatggttgggctttttctcaaagggtctaactgagggcttgagcgaccttgagataactgtgtttttagagatcttgtatcctgtgtaaaggcagaaccaaccgcactactttggggtaaggtaccactgtttgatgtttctgttccaaaggatgtcaaagagcttccagcaacaccaacagcaccaaactgctgcccaactaaggaactcggactgaactgactgtatgtgggcatcctgccgaaaggtccataagaacccatggactggaatgaagaagtcgatgagcctagtgaggacatcagttacctgaacaatagctgggtcttgaggcaaagaacactgtggttttggtggctcacaaacagtaaggtctttaatgtcactcccacggaatataatgtattcaaagacttcatctcgaggtggtattggacgatctgtcggtctgtcttctgtaccaaaggatcgaactttggcaagggctacggtggagttttcggtgtcgatggtgtagaggatgccctcgtagcggatctccgccttggagatgaggctgatcttgctgccgatgtaaggggtgcccccgctcatggcgccgccgccgccgctcccagctgctcgcagagaggcagatcccacgccactgtcgcccgctccgcacgcccgctcgctccgtcggcgcctacagcagccgcttcagacccaacatggcggcggcgccggctccgct

SEQ ID NO: 9658 - RNA, 1995 nt, Homo sapiens
  source 1..1995: mol_type = other RNA
atcccacctctgccaccaccacgccctctgccaccacggaaaccaagacctcctctgcctctgtatcccccacggccacggtttggacgaagtgggattccaaatgtttcagcatttaatcttctttcttcagcccaggttggtctccgttctctattgtcatcacaagaaatattatcaaagaaggatttagttttgtcataatagcaattaggtccaagtggatcttcttcatcggcatttccttcactgttttgggtatcaactcctgagtctcctttatcttcaccatttacaggcttctcctgtttctcaagtttatcttcttttaatttaagtttattatgaaactctctgtcaatctcttccttgttgaattgtgcatttgcactttcaaagtcaaagtctttctcaaatttcattggcccatctcgccgaataccaaatcttcccctgccaccccgatgacccccacgccctctccttggagctgaaggagcacctggagctacttgtctcttgttatcatttctgagttgctcattttctggccttgaaactttgtgtacttcagctcgcctgtgctcctgattctctcctgccttttggctggcagatggcaaaggcctggttgatacaggactccttctcccaacagctgctggagcaggtaagtgggctgaggcggtctgcactgcttgttccatggttgggctttttctcaaagggtctaactgagggcttgagcgaccttgagataactgtgtttttagagatcttgtatcctgtgtaaaggcagaaccaaccgcactactttggggtaaggtaccactgtttgatgtttctgttccaaaggatgtcaaagagcttccagcaacaccaacagcaccaaactgctgcccaactaaggaactcggactgaactgactgtatgtgggcatcctgccgaaaggtccataagaacccatggactggaatgaagaagtcgatgagcctagtgaggactgaacaatagctgggtcttgaggcaaagaacactgtggttttggtggctcacaaacagtaaggtctttaatgtcactcccacggaatataatgtattcaaagacttcatctcgaggtggtattggacgatctgtcggtctgtcttctgtaccaaaggatcgaacaacagaggatgagccgagggagatgggatctgctccacggcatcgatggcatttcgagaatgtctgcgtcgcagagcaaacccaaagttttagcacattactcaagagttcaccagaggaagatcgccacgaattgaaatgaacaaagtgagaaaatgggtgctgtgtagtcaacgcatccgcgatgaactcaagctgggcggaaaaattctttgaatactccggctttgttttgtgctaagacggcagaagccccgaatttcggagttggaagacgcgtttctccgtgttctccggcccgttctcggacttcagggccgcccgccgcgcactcagtcccgtagttccccgggcttcaggcgcggacattccggggggcggaaaccagggagccgcggggaggccgcggtccggcccgcgacgccggggcccggagaagggaggcgagaggcctcccggagctcgacggagggaggggagggaacgaggaggccgcgggccggagcggggagcagccccgagcggcgcccggctcggcccccaccctgaggcccggtcccgcgtacctttggcaagggctacggtggagttttcggtgtcgatggtgtagaggatgccctcgtagcggatctccgccttggagatgaggctgatcttgctgccgatgtaaggggtgcccccgctcatggcgccgccgccgccgctcccagctgctcgcagagaggcagatcccacgccactgtcgcccgctccgcacgcccgctcgctccgtcggcgcctacagcagccgcttcagacccaacatggcggcggcgccggctccgct

SEQ ID NO: 9659 - RNA, 2137 nt, Homo sapiens
  source 1..2137: mol_type = other RNA
atcccacctctgccaccaccacgccctctgccaccacggaaaccaagacctcctctgcctctgtatcccccacggccacggtttggacgaagtgggattccaaatgtttcagcatttaatcttctttcttcagcccaggttggtctccgttctctattgtcatcacaagaaatattatcaaagaaggatttagttttgtcataatagcaattaggtccaagtggatcttcttcatcggcatttccttcactgttttgggtatcaactcctgagtctcctttatcttcaccatttacaggcttctcctgtttctcaagtttatcttcttttaatttaagtttattatgaaactctctgtcaatctcttccttgttgaattgtgcatttgcactttcaaagtcaaagtctttctcaaatttcattggcccatctcgccgaataccaaatcttcccctgccaccccgatgacccccacgccctctccttggagctgaaggagcacctggagctacttgtctcttgttatcatttctgagttgctcattttctggccttgaaactttgtgtacttcagctcgcctgtgctcctgattctctcctgccttttggctggcagatggcaaaggcctggttgatacaggactccttctcccaacagctgctggagcaggtaagtgggctgaggcggtctgcactgcttgttccatggttgggctttttctcaaagggtctaactgagggcttgagcgaccttgagataactgtgtttttagagatcttgtatcctgtgtaaaggcagaaccaaccgcactactttggggtaaggtaccactgtttgatgtttctgttccaaaggatgtcaaagagcttccagcaacaccaacagcaccaaactgctgcccaactaaggaactcggactgaactgactgtatgtgggcatcctgccgaaaggtccataagaacccatggactggaatgaagaagtcgatgagcctagtgaggactgaacaatagctgggtcttgaggcaaagaacactgtggttttggtggctcacaaacagtaaggtctttaatgtcactcccacggaatataatgtattcaaagacttcatctcgaggtggtattggacgatctgtcggtctgtcttctgtaccaaaggatcgaactggtcaagaaggatcctggatcaagcttgaacccgtttccagaaacaggggcgtcggggcagcagcaagcatttttaccacgcgccctaatgaggtggttgcacaacaggctttgaggattccggtttaacaggtaaataccaacagaggatgagccgagggagatgggatctgctccacggcatcgatggcatttcgagaatgtctgcgtcgcagagcaaacccaaagttttagcacattactcaagagttcaccagaggaagatcgccacgaattgaaatgaacaaagtgagaaaatgggtgctgtgtagtcaacgcatccgcgatgaactcaagctgggcggaaaaattctttgaatactccggctttgttttgtgctaagacggcagaagccccgaatttcggagttggaagacgcgtttctccgtgttctccggcccgttctcggacttcagggccgcccgccgcgcactcagtcccgtagttccccgggcttcaggcgcggacattccggggggcggaaaccagggagccgcggggaggccgcggtccggcccgcgacgccggggcccggagaagggaggcgagaggcctcccggagctcgacggagggaggggagggaacgaggaggccgcgggccggagcggggagcagccccgagcggcgcccggctcggcccccaccctgaggcccggtcccgcgtacctttggcaagggctacggtggagttttcggtgtcgatggtgtagaggatgccctcgtagcggatctccgccttggagatgaggctgatcttgctgccgatgtaaggggtgcccccgctcatggcgccgccgccgccgctcccagctgctcgcagagaggcagatcccacgccactgtcgcccgctccgcacgcccgctcgctccgtcggcgcctacagcagccgcttcagacccaacatggcggcggcgccggctccgct

SEQ ID NO: 9660 - RNA, 1546 nt, Homo sapiens
  source 1..1546: mol_type = other RNA
atcccacctctgccaccaccacgccctctgccaccacggaaaccaagacctcctctgcctctgtatcccccacggccacggtttggacgaagtgggattccaaatgtttcagcatttaatcttctttcttcagcccaggttggtctccgttctctattgtcatcacaagaaatattatcaaagaaggatttagttttgtcataatagcaattaggtccaagtggatcttcttcatcggcatttccttcactgttttgggtatcaactcctgagtctcctttatcttcaccatttacaggcttctcctgtttctcaagtttatcttcttttaatttaagtttattatgaaactctctgtcaatctcttccttgttgaattgtgcatttgcactttcaaagtcaaagtctttctcaaatttcattggcccatctcgccgaataccaaatcttcccctgccaccccgatgacccccacgccctctccttggagctgaaggagcacctggagctacttgtctcttgttatcatttctgagttgctcattttctggccttgaaactttgtgtacttcagctcgcctgtgctcctgattctctcctgccttttggctggcagatggcaaaggcctggttgatacaggactccttctcccaacagctgctggagcaggtaagtgggctgaggcggtctgcactgcttgttccatggttgggctttttctcaaagggtctaactgagggcttgagcgaccttgagataactgtgtttttagagatcttgtatcctgtgtaaaggcagaaccaaccgcactactttggggtaaggtaccactgtttgatgtttctgttccaaaggatgtcaaagagcttccagcaacaccaacagcaccaaactgctgcccaactaaggaactcggactgaactgactgtatgtgggcatcctgccgaaaggtccataagaacccatggactggaatgaagaagtcgatgagcctagtgaggactgaacaatagctgggtcttgaggcaaagaacactgtggttttggtggctcacaaacagtaaggtctttaatgtcactcccacggaatataatgtattcaaagacttcatctcgaggtggtattggacgatctgtcggtctgtcttctgtaccaaaggatcgaactgtagtcctagctgctcaggtggctgaggcgggaggattggctgaactcaagaggcagaagttgcagtgagccaagatggcgctcctgcactccagcctgggtgacagaatgacaatctttggcaagggctacggtggagttttcggtgtcgatggtgtagaggatgccctcgtagcggatctccgccttggagatgaggctgatcttgctgccgatgtaaggggtgcccccgctcatggcgccgccgccgccgctcccagctgctcgcagagaggcagatcccacgccactgtcgcccgctccgcacgcccgctcgctccgtcggcgcctacagcagccgcttcagacccaacatggcggcggcgccggctccgct

SEQ ID NO: 9661 - RNA, 1428 nt, Homo sapiens
  source 1..1428: mol_type = other RNA
atcccacctctgccaccaccacgccctctgccaccacggaaaccaagacctcctctgcctctgtatcccccacggccacggtttggacgaagtgggattccaaatgtttcagcatttaatcttctttcttcagcccaggttggtctccgttctctattgtcatcacaagaaatattatcaaagaaggatttagttttgtcataatagcaattaggtccaagtggatcttcttcatcggcatttccttcactgttttgggtatcaactcctgagtctcctttatcttcaccatttacaggcttctcctgtttctcaagtttatcttcttttaatttaagtttattatgaaactctctgtcaatctcttccttgttgaattgtgcatttgcactttcaaagtcaaagtctttctcaaatttcattggcccatctcgccgaataccaaatcttcccctgccaccccgatgacccccacgccctctccttggagctgaaggagcacctggagctacttgtctcttgttatcatttctgagttgctcattttctggccttgaaactttgtgtacttcagctcgcctgtgctcctgattctctcctgccttttggctggcagatggcaaaggcctggttgatacaggactccttctcccaacagctgctggagcaggtaagtgggctgaggcggtctgcactgcttgttccatggttgggctttttctcaaagggtctaactgagggcttgagcgaccttgagataactgtgtttttagagatcttgtatcctgtgtaaaggcagaaccaaccgcactactttggggtaaggtaccactgtttgatgtttctgttccaaaggatgtcaaagagcttccagcaacaccaacagcaccaaactgctgcccaactaaggaactcggactgaactgactgtatgtgggcatcctgccgaaaggtccataagaacccatggactggaatgaagaagtcgatgagcctagtgaggactgaacaatagctgggtcttgaggcaaagaacactgtggttttggtggctcacaaacagtaaggtctttaatgtcactcccacggaatataatgtattcaaagacttcatctcgaggtggtattggacgatctgtcggtctgtcttctgtaccaaaggatcgaactttggcaagggctacggtggagttttcggtgtcgatggtgtagaggatgccctcgtagcggatctccgccttggagatgaggctgatcttgctgccgatgtaaggggtgcccccgctcatggcgccgccgccgccgctcccagctgctcgcagagaggcagatcccacgccactgtcgcccgctccgcacgcccgctcgctccgtcggcgcctacagcagccgcttcagacccaacatggcggcggcgccggctccgct

SEQ ID NO: 9662 - RNA, 1433 nt, Homo sapiens
  source 1..1433: mol_type = other RNA
atcccacctctgccaccaccacgccctctgccaccacggaaaccaagacctcctctgcctctgtatcccccacggccacggtttggacgaagtgggattccaaatgtttcagcatttaatcttctttcttcagcccaggttggtctccgttctctattgtcatcacaagaaatattatcaaagaaggatttagttttgtcataatagcaattaggtccaagtggatcttcttcatcggcatttccttcactgttttgggtatcaactcctgagtctcctttatcttcaccatttacaggcttctcctgtttctcaagtttatcttcttttaatttaagtttattatgaaactctctgtcaatctcttccttgttgaattgtgcatttgcactttcaaagtcaaagtctttctcaaatttcattggcccatctcgccgaataccaaatcttcccctgccaccccgatgacccccacgccctctccttggagctgaaggagcacctggagctacttgtctcttgttatcatttctgagttgctcattttctggccttgaaactttgtgtacttcagctcgcctgtgctcctgattctctcctgccttttggctggcagatggcaaaggcctggttgatacaggactccttctcccaacagctgctggagcaggtaagtgggctgaggcggtctgcactgcttgttccatggttgggctttttctcaaagggtctaactgagggcttgagcgaccttgagataactgtgtttttagagatcttgtatcctgtgtaaaggcagaaccaaccgcactactttggggtaaggtaccactgtttgatgtttctgttccaaaggatgtcaaagagcttccagcaacaccaacagcaccaaactgctgcccaactaaggaactcggactgaactgactgtatgtgggcatcctgccgaaaggtccataagaacccatggactggaatgaagaagtcgatgagcctagtgaggactgaacaatagctgggtcttgaggcaaagaacactgtggttttggtggctcacaaacagtaaggtctttaatgtcactcccacggaatataatgtattcaaagacttcatctcgaggtggtattggacgatctgtcggtctgtcttctgtaccaaaggatcgaactttggcaagggctacggtggagttttcggtgtcgatggtgtagaggatgccctcgtagcggatctccgccttggagatgaggctgatcttgctgccgatgtaaggggtgcccccgctcatggcgccgccgccgccgctcccagctgctcgcagagaggcagatcccacgccactgtcgcccgctccgcacgcccgctcgctccgtcggcgcctacagcagccgcttcagacccaacatggcggcggcgccggctccgctaccct

SEQ ID NO: 9663 - RNA, 1530 nt, Homo sapiens
  source 1..1530: mol_type = other RNA
atcccacctctgccaccaccacgccctctgccaccacggaaaccaagacctcctctgcctctgtatcccccacggccacggtttggacgaagtgggattccaaatgtttcagcatttaatcttctttcttcagcccaggttggtctccgttctctattgtcatcacaagaaatattatcaaagaaggatttagttttgtcataatagcaattaggtccaagtggatcttcttcatcggcatttccttcactgttttgggtatcaactcctgagtctcctttatcttcaccatttacaggcttctcctgtttctcaagtttatcttcttttaatttaagtttattatgaaactctctgtcaatctcttccttgttgaattgtgcatttgcactttcaaagtcaaagtctttctcaaatttcattggcccatctcgccgaataccaaatcttcccctgccaccccgatgacccccacgccctctccttggagctgaaggagcacctggagctacttgtctcttgttatcatttctgagttgctcattttctggccttgaaactttgtgtacttcagctcgcctgtgctcctgattctctcctgccttttggctggcagatggcaaaggcctggttgatacaggactccttctcccaacagctgctggagcaggtaagtgggctgaggcggtctgcactgcttgttccatggttgggctttttctcaaagggtctaactgagggcttgagcgaccttgagataactgtgtttttagagatcttgtatcctgtgtaaaggcagaaccaaccgcactactttggggtaaggtaccactgtttgatgtttctgttccaaaggatgtcaaagagcttccagcaacaccaacagcaccaaactgctgcccaactaaggaactcggactgaactgactgtatgtgggcatcctgccgaaaggtccataagaacccatggactggaatgaagaagtcgatgagcctagtgaggactgtaatcccagctactcaggaggctgaggcagaagaatcacttgaacctgggaggcggaggttgtagtgagccgagttcacgccactgtactccaacgactctgaacaatagctgggtcttgaggcaaagaacactgtggttttggtggctcacaaacagtaaggtctttaatgtcactcccacggaatataatgtattcaaagacttcatctcgaggtggtattggacgatctgtcggtctgtcttctgtaccaaaggatcgaactttggcaagggctacggtggagttttcggtgtcgatggtgtagaggatgccctcgtagcggatctccgccttggagatgaggctgatcttgctgccgatgtaaggggtgcccccgctcatggcgccgccgccgccgctcccagctgctcgcagagaggcagatcccacgccactgtcgcccgctccgcacgcccgctcgctccgtcggcgcctacagcagccgcttcagacccaacatggcggcggcgccggctccgct

SEQ ID NO: 9664 - RNA, 1494 nt, Homo sapiens
  source 1..1494: mol_type = other RNA
atcccacctctgccaccaccacgccctctgccaccacggaaaccaagacctcctctgcctctgtatcccccacggccacggtttggacgaagtgggattccaaatgtttcagcatttaatcttctttcttcagcccaggttggtctccgttctctattgtcatcacaagaaatattatcaaagaaggatttagttttgtcataatagcaattaggtccaagtggatcttcttcatcggcatttccttcactgttttgggtatcaactcctgagtctcctttatcttcaccatttacaggcttctcctgtttctcaagtttatcttcttttaatttaagtttattatgaaactctctgtcaatctcttccttgttgaattgtgcatttgcactttcaaagtcaaagtctttctcaaatttcattggcccatctcgccgaataccaaatcttcccctgccaccccgatgacccccacgccctctccttggagctgaaggagcacctggagctacttgtctcttgttatcatttctgagttgctcattttctggccttgaaactttgtgtacttcagctcgcctgtgctcctgattctctcctgccttttggctggcagatggcaaaggcctggttgatacaggactccttctcccaacagctgctggagcaggtaagtgggctgaggcggtctgcactgcttgttccatggttgggctttttctcaaagggtctaactgagggcttgagcgaccttgagataactgtgtttttagagatcttgtatcctgtgtaaaggcagaaccaaccgcactactttggggtaaggtaccactgtttgatgtttctgttccaaaggatgtcaaagagcttccagctcttctctcaacattttctatattttcaccagtctagcccacagcagaagtttatccttctgctccaacaccaacagcaccaaactgctgcccaactaaggaactcggactgaactgactgtatgtgggcatcctgccgaaaggtccataagaacccatggactggaatgaagaagtcgatgagcctagtgaggactgaacaatagctgggtcttgaggcaaagaacactgtggttttggtggctcacaaacagtaaggtctttaatgtcactcccacggaatataatgtattcaaagacttcatctcgaggtggtattggacgatctgtcggtctgtcttctgtaccaaaggatcgaactttggcaagggctacggtggagttttcggtgtcgatggtgtagaggatgccctcgtagcggatctccgccttggagatgaggctgatcttgctgccgatgtaaggggtgcccccgctcatggcgccgccgccgccgctcccagctgctcgcagagaggcagatcccacgccactgtcgcccgctccgcacgcccgctcgctccgtcggcgcctacagcagccgcttcagacccaacatggcggcggcgccggctccgct

SEQ ID NO: 9665 - RNA, 1512 nt, Homo sapiens
  source 1..1512: mol_type = other RNA
atcccacctctgccaccaccacgccctctgccaccacggaaaccaagacctcctctgcctctgtatcccccacggccacggtttggacgaagtgggattccaaatgtttcagcatttaatcttctttcttcagcccaggttggtctccgttctctattgtcatcacaagaaatattatcaaagaaggatttagttttgtcataatagcaattaggtccaagtggatcttcttcatcggcatttccttcactgttttgggtatcaactcctgagtctcctttatcttcaccatttacaggcttctcctgtttctcaagtttatcttcttttaatttaagtttattatgaaactctctgtcaatctcttccttgttgaattgtgcatttgcactttcaaagtcaaagtctttctcaaatttcattggcccatctcgccgaataccaaatcttcccctgccaccccgatgacccccacgccctctccttggagctgaaggagcacctggagctacttgtctcttgttatcatttctgagttgctcattttctggccttgaaactttgtgtacttcagctcgcctgtgctcctgattctctcctgccttttggctggcagatggcaaaggcctggttgatacaggactccttctcccaacagctgctggagcaggtaagtgggctgaggcggtctgcactgcttgttccatggttgggctttttctcaaagggtctaactgagggcttgagcgaccttgagataactgtgtttttagagatcttgtatcctgtgtaaaggcagaaccaaccgcactactttggggtaaggtaccactgtttgatgtttctgttccaaaggatgtcaaagagcttccagctttcccattccatatttatatcttccgtctccatggtaaaaacactatttcccaacataagtattttattcatttgccctttccaacaccaacagcaccaaactgctgcccaactaaggaactcggactgaactgactgtatgtgggcatcctgccgaaaggtccataagaacccatggactggaatgaagaagtcgatgagcctagtgaggactgaacaatagctgggtcttgaggcaaagaacactgtggttttggtggctcacaaacagtaaggtctttaatgtcactcccacggaatataatgtattcaaagacttcatctcgaggtggtattggacgatctgtcggtctgtcttctgtaccaaaggatcgaactttggcaagggctacggtggagttttcggtgtcgatggtgtagaggatgccctcgtagcggatctccgccttggagatgaggctgatcttgctgccgatgtaaggggtgcccccgctcatggcgccgccgccgccgctcccagctgctcgcagagaggcagatcccacgccactgtcgcccgctccgcacgcccgctcgctccgtcggcgcctacagcagccgcttcagacccaacatggcggcggcgccggctccgct

SEQ ID NO: 9666 - RNA, 1251 nt, Homo sapiens
  source 1..1251: mol_type = other RNA
atcccacctctgccaccaccacgccctctgccaccacggaaaccaagacctcctctgcctctgtatcccccacggccacggtttggacgaagtgggattccaaatgtttcagcatttaatcttctttcttcagcccaggttggtctccgttctctattgtcatcacaagaaatattatcaaagaaggatttagttttgtcataatagcaattaggtccaagtggatcttcttcatcggcatttccttcactgttttgggtatcaactcctgagtctcctttatcttcaccatttacaggcttctcctgtttctcaagtttatcttcttttaatttaagtttattatgaaactctctgtcaatctcttccttgttgaattgtgcatttgcactttcaaagtcaaagtctttctcaaatttcattggcccatctcgccgaataccaaatcttcccctgccaccccgatgacccccacgccctctccttggagctgaaggagcacctggagctacttgtctcttgttatcatttctgagttgctcattttctggccttgaaactttgtgtacttcagcttgagataactgtgtttttagagatcttgtatcctgtgtaaaggcagaaccaaccgcactactttggggtaaggtaccactgtttgatgtttctgttccaaaggatgtcaaagagcttccagcaacaccaacagcaccaaactgctgcccaactaaggaactcggactgaactgactgtatgtgggcatcctgccgaaaggtccataagaacccatggactggaatgaagaagtcgatgagcctagtgaggactgaacaatagctgggtcttgaggcaaagaacactgtggttttggtggctcacaaacagtaaggtctttaatgtcactcccacggaatataatgtattcaaagacttcatctcgaggtggtattggacgatctgtcggtctgtcttctgtaccaaaggatcgaactttggcaagggctacggtggagttttcggtgtcgatggtgtagaggatgccctcgtagcggatctccgccttggagatgaggctgatcttgctgccgatgtaaggggtgcccccgctcatggcgccgccgccgccgctcccagctgctcgcagagaggcagatcccacgccactgtcgcccgctccgcacgcccgctcgctccgtcggcgcctacagcagccgcttcagacccaacatggcggcggcgccggctccgct

SEQ ID NO: 9667 - RNA, 1256 nt, Homo sapiens
  source 1..1256: mol_type = other RNA
atcccacctctgccaccaccacgccctctgccaccacggaaaccaagacctcctctgcctctgtatcccccacggccacggtttggacgaagtgggattccaaatgtttcagcatttaatcttctttcttcagcccaggttggtctccgttctctattgtcatcacaagaaatattatcaaagaaggatttagttttgtcataatagcaattaggtccaagtggatcttcttcatcggcatttccttcactgttttgggtatcaactcctgagtctcctttatcttcaccatttacaggcttctcctgtttctcaagtttatcttcttttaatttaagtttattatgaaactctctgtcaatctcttccttgttgaattgtgcatttgcactttcaaagtcaaagtctttctcaaatttcattggcccatctcgccgaataccaaatcttcccctgccaccccgatgacccccacgccctctccttggagctgaaggagcacctggagctacttgtctcttgttatcatttctgagttgctcattttctggccttgaaactttgtgtacttcagcttgagataactgtgtttttagagatcttgtatcctgtgtaaaggcagaaccaaccgcactactttggggtaaggtaccactgtttgatgtttctgttccaaaggatgtcaaagagcttccagcaacaccaacagcaccaaactgctgcccaactaaggaactcggactgaactgactgtatgtgggcatcctgccgaaaggtccataagaacccatggactggaatgaagaagtcgatgagcctagtgaggactgaacaatagctgggtcttgaggcaaagaacactgtggttttggtggctcacaaacagtaaggtctttaatgtcactcccacggaatataatgtattcaaagacttcatctcgaggtggtattggacgatctgtcggtctgtcttctgtaccaaaggatcgaactttggcaagggctacggtggagttttcggtgtcgatggtgtagaggatgccctcgtagcggatctccgccttggagatgaggctgatcttgctgccgatgtaaggggtgcccccgctcatggcgccgccgccgccgctcccagctgctcgcagagaggcagatcccacgccactgtcgcccgctccgcacgcccgctcgctccgtcggcgcctacagcagccgcttcagacccaacatggcggcggcgccggctccgctaccct

SEQ ID NO: 9668 - RNA, 1185 nt, Homo sapiens
  source 1..1185: mol_type = other RNA
atcccacctctgccaccaccacgccctctgccaccacggaaaccaagacctcctctgcctctgtatcccccacggccacggtttggacgaagtgggattccaaatgtttcagcatttaatcttctttcttcagcccaggttggtctccgttctctattgtcatcacaagaaatattatcaaagaaggatttagttttgtcataatagcaattaggtccaagtggatcttcttcatcggcatttccttcactgttttgggtatcaactcctgagtctcctttatcttcaccatttacaggcttctcctgtttctcaagtttatcttcttttaatttaagtttattatgaaactctctgtcaatctcttccttgttgaattgtgcatttgcactttcaaagtcaaagtctttctcaaatttcattggcccatctcgccgaataccaaatcttcccctgccaccccgatgacccccacgccctctccttggagctgaaggagcacctggagcttgagataactgtgtttttagagatcttgtatcctgtgtaaaggcagaaccaaccgcactactttggggtaaggtaccactgtttgatgtttctgttccaaaggatgtcaaagagcttccagcaacaccaacagcaccaaactgctgcccaactaaggaactcggactgaactgactgtatgtgggcatcctgccgaaaggtccataagaacccatggactggaatgaagaagtcgatgagcctagtgaggactgaacaatagctgggtcttgaggcaaagaacactgtggttttggtggctcacaaacagtaaggtctttaatgtcactcccacggaatataatgtattcaaagacttcatctcgaggtggtattggacgatctgtcggtctgtcttctgtaccaaaggatcgaactttggcaagggctacggtggagttttcggtgtcgatggtgtagaggatgccctcgtagcggatctccgccttggagatgaggctgatcttgctgccgatgtaaggggtgcccccgctcatggcgccgccgccgccgctcccagctgctcgcagagaggcagatcccacgccactgtcgcccgctccgcacgcccgctcgctccgtcggcgcctacagcagccgcttcagacccaacatggcggcggcgccggctccgct

SEQ ID NO: 9669 - RNA, 1424 nt, Homo sapiens
  source 1..1424: mol_type = other RNA
atcccacctctgccaccaccacgccctctgccaccacggaaaccaagacctcctctgcctctgtatcccccacggccacggtttggacgaagtgggattccaaatgtttcagcatttaatcttctttcttcagcccaggttggtctccgttctctattgtcatcacaagaaatattatcaaagaaggatttagttttgtcataatagcaattaggtccaagtggatcttcttcatcggcatttccttcactgttttgggtatcaactcctgagtctcctttatcttcaccatttacaggcttctcctgtttctcaagtttatcttcttttaatttaagtttattatgaaactctctgtcaatctcttccttgttgaattgtgcatttgcactttcaaagtcaaagtctttctcaaatttcattggcccatctcgccgaataccaaatcttcccctgccaccccgatgacccccacgccctctccttggagctgaaggagcacctggagttgtctcttgttatcatttctgagttgctcattttctggccttgaaactttgtgtacttcagctcgcctgtgctcctgattctctcctgccttttggctggcagatggcaaaggcctggttgatacaggactccttctcccaacagctgctggagcaggtaagtgggctgaggcggtctgcactgcttgttccatggttgggctttttctcaaagggtctaactgagggcttgagcgaccttgagataactgtgtttttagagatcttgtatcctgtgtaaaggcagaaccaaccgcactactttggggtaaggtaccactgtttgatgtttctgttccaaaggatgtcaaagagcttccagcaacaccaacagcaccaaactgctgcccaactaaggaactcggactgaactgactgtatgtgggcatcctgccgaaaggtccataagaacccatggactggaatgaagaagtcgatgagcctagtgaggactgaacaatagctgggtcttgaggcaaagaacactgtggttttggtggctcacaaacagtaaggtctttaatgtcactcccacggaatataatgtattcaaagacttcatctcgaggtggtattggacgatctgtcggtctgtcttctgtaccaaaggatcgaactttggcaagggctacggtggagttttcggtgtcgatggtgtagaggatgccctcgtagcggatctccgccttggagatgaggctgatcttgctgccgatgtaaggggtgcccccgctcatggcgccgccgccgccgctcccagctgctcgcagagaggcagatcccacgccactgtcgcccgctccgcacgcccgctcgctccgtcggcgcctacagcagccgcttcagacccaacatggcggcggcgccggctccgct

SEQ ID NO: 9670 - RNA, 492 nt, Homo sapiens
  source 1..492: mol_type = other RNA
atccgcgctctgactctctgcctctcctcaggtctcccattcacatgtccctcagaaaatcttccatgtcgttttcatgtaaagatgtatgtccctctatttatgatgtatcagaatctcttaaggtgtgtgggtagagaatttggaaggaaacctgagctgatcatactgtgcattctttgctgagccaagagctgctctcgtccagccaccccatctgtgtgcaaagcagaaaggacagagtggatgctatagctctctggagtttaggttatcccggaaactacaagcaggtgggaaataggaacgtgcttcggggttatttctttgtcagaatacgtagaaaattattaagtctacccacgagaaaaagaaaccaattaaacctggcttagagttcttcaggctgctagggttttgttgcaaaaaccctcagtcctgcaagtggctccagccggtgcccttctcctatctgtgtctgtgcctctcttc

SEQ ID NO: 9671 - RNA, 1910 nt, Homo sapiens
  source 1..1910: mol_type = other RNA
atcctctcttccctcctcccagcgcactctccttccagtaaaaagtggttaaagggacagcgccatcaatttcccagctctgagggtctgcttagaactagggggctggaaggagacagagggcaaagagaaaggaactggcagaggtctttcctgggggatatgtctgttctgtcctggggatcctggagcaggaaaacccgcgtaaagtaggggtgtagtgggtgttgagataactgcctgggggaggttcagagtggaagtacgagtctacaaactctcaagggcgtctcagggctcccagcatccccaggggtcctttcgcaggggtccctaagcaggaggggaacagcccagaaaacacggaactggacccccgacaggaagtccagggaggggtccctggctcactatgtgaccctgctggatcacttgcctcccctctcgggtcccctcagcacagtgtccctcccttccttcccctaaagtaaaagcagagggttaatctctttccccgccccacgcccaacaaagagcaggccctgtccccggtgctgaagcgccagccgcagcaccacccccactcccacagcataaaacatgagccaaaaccaataaagagccaaatgtcacagccgttgcagggccccctaaatcctggggaccccttcttctacctgacatcctattggggtgagggactttggtactcagaaagcatctcatcacttccctgtaagagagaagggatgccgactcaggcgcctgcttgtctgttacaggagtgggggaagagaggacaagttgaggctgagaagatggggagggggagggagaaaagaggacttcctagtgttgacagaacggcaagatgtgggttccccatccccagttcagccagagacccctcaaagtggaacttcctggggcagtcgggggtcaggagttggagcttgtctctggggcaagaccccttcgttgtacagatggaaaaacaagggtgggaggacacagcttgtccaaggtcattcgaccagcaaactgcctagctgaccccagtgtgcagaagctggctcgggtgacacccatcatttccccccaccccacacaggggccagctctctcaacttcatgcccaagccctcctacggtacccccactgtaggttctctgcccctcaaactcagcccagctttctcctgcctgttcaggggaccttctgcccgcttcgctgagggtccgtcccctttactggggctggcagcagggtctcccatctcctctctcgggggccactgcagactttttagagaacgccttgcctccccccaaccccacccatccggggttccctctctccatcctctgcagtgtctcccatacccccattcagggtagccttgctattctccccaactccaggtcccccttcatctattccggggctggccgcggagtttcctgagcgctctccaagtgggtcctctagatgttaggagaacactgtacctcccccggtcaggggtctcctgtctccgttctatggagcgtccatgctcccattcaggactgccttgctccctcctctgttccggggctggctgcacagtctctgcaccccctatcctgaaagcctctcttaactatttggaaagcctcgtgtcctgtctcatacagggatcccctcatcctaatgactgcaatcttccattgctccatcccgagggcatcctgcccctattcccatcaggtttctccttgtcctctccctgtttcaagtcccctttcttattccgaacacactcgcaggctcttccgacgcgcacccgggggtcctcactggcccactccgggagtcctctgcccgcttccccgacctcgagggtctcctctgacgcagcgtcgattcc

SEQ ID NO: 9672 - RNA, 243 nt, Homo sapiens
  source 1..243: mol_type = other RNA
atcctctcttccctcctcccaggaggcctgtcctcatttcaaagcagttcacagccaccttatcgcctgaaagcctgctcctcttctccgtcactgttgtctcccagccctttctcactggtgtttgcaatccttctcggcttcactcagtctgtgagcttgttcctgacatctggaatggcagctcactggagccactctgctgtcagcatcctgctccacgctggctgcagtgaagctgtg

SEQ ID NO: 9673 - RNA, 240 nt, Homo sapiens
  source 1..240: mol_type = other RNA
atcctctcttccctcctcccaggcacagcagcccggcccagcttccgtggctatgaaatcgcttccgggttcacaccctttgcagcctcgcggttggcggtgaaagagcttccgggtcggcggccgggctgctgccgttcctgctccttttcactggacctgcagtctctcaggggctggtggcaggcgactaggagactagggtggtggcggtgggggtgccagcggctgagccggagc

SEQ ID NO: 9674 - RNA, 356 nt, Homo sapiens
  source 1..356: mol_type = other RNA
atcctctcttccctcctcccaggcacagcagcccggcccagcttcctgctctttactgtccttccctctcctcgcacctcagcaccattcacccctcaccctctcccgaaactacggggtcccaggtcttcaaaggccttagctttccaccccgccgttaccgtggctatgaaatcgcttccgggttcacaccctttgcagcctcgcggttggcggtgaaagagcttccgggtcggcggccgggctgctgccgttcctgctccttttcactggacctgcagtctctcaggggctggtggcaggcgactaggagactagggtggtggcggtgggggtgccagcggctgagccggagc

SEQ ID NO: 9675 - RNA, 469 nt, Homo sapiens
  source 1..469: mol_type = other RNA
atcctctcttccctcctcccaggcacagcagcccggcccagcttcctgtggcagaaaaaccctcagtcgccaaaagaaagccgtcttgagggttcccccgcgctcccacccgcgccccaaaagctcaggtctctggagtcggagaccctcctgcccacctgctctttactgtccttccctctcctcgcacctcagcaccattcacccctcaccctctcccgaaactacggggtcccaggtcttcaaaggccttagctttccaccccgccgttaccgtggctatgaaatcgcttccgggttcacaccctttgcagcctcgcggttggcggtgaaagagcttccgggtcggcggccgggctgctgccgttcctgctccttttcactggacctgcagtctctcaggggctggtggcaggcgactaggagactagggtggtggcggtgggggtgccagcggctgagccggagc

SEQ ID NO: 9676 - RNA, 1265 nt, Homo sapiens
  source 1..1265: mol_type = other RNA
atcctctcttccctcctcccagggctggcatgctggccggaaagctccagcagctgggtccttgggcatcttgtcagcatctctgtgggatcactgcagacatttctccagcatagaggcttcagggtggccaggttttttgcatgatggccaaagcctctgaaggccatgtccctggcctctgatgtggctgacggctcagttatctgcttggagagagctccacgtccactagaaagaatgagggctttgcagtgtcactcaggtcaggtgatggtcacgttccttcagggcctcttggtctggatcagggctttgcaatgctggagacagaagctgctgacagtgaggagtccttcaggctctttgaggtcacaatcttccatgatgtggccctggcctccagaaaggttcttctgcgcagcatctattccgagaacaagaaagaagttctcctggcaacgggactcgctccagaggcgctgagaagtagacgtggtgtgtatgctctgaagggctctccagagttttctggattcgttacacaatttatgtacacgttcaacgccaggtttttcttcactgcttatttctaggaaatggtctatggtggaaacgtcttcagctgcctgctggactgttatttcttgaaaagcacactttaaaatgttctcatagctgagaatgggctcagaaggtgggacggcagaagttcctgtcacccaaggtccaccctggcatggttggtgagaactgcactcttttggggcagaagtggttctcggtggctggggttctgtgggtccctcgaggagttcaagggactgtgagaattgtccagacttggctgaagattcccgaaagccttcaaactccccccaagtgctgctgtgttccccagggtcaggacatcgggcagtgcaggtggaaccgccctcacggggcatggagatgctggctttcccatcggacaggagaaggtcggggcaggtccgtctccattccaaactgtcatcactcagcctctcaggtgccactcggagggaagcgctggctgcttcctcctggaggtcactcaaaggctctccccccagctcccgccggccttgcatcttggagcccccaggccagcagaggcccgatgggcagctgctcaggagacatgcacgccggggtgctggccgcccaggactgcccaaccttcccctgccctggagagggccaggggacgctgcaggagtgccccgggctgcccagtggctgac

SEQ ID NO: 9677 - RNA, 1424 nt, Homo sapiens
  source 1..1424: mol_type = other RNA
atccttgctatctgggtgctaagcacctcctccaccgacatgcccgggaagaggttggtcatcagcagggacagctttggttgcttggggttgaggagcaggacagtggccacatcctggcgggccccaaaaatgttctgcagcagctgccggctcttggcccggtacaggtagtactgggccttctgggggttgtgccggatggccgtggagaagtggttctctgccttctggaactgccgcctcggttgatgtagagtcctttctcctgctgctcgtcccggagggccttgttcagcagcagcacgccctcctggtaggcgccctgcctgtagcagtgcacggcaaagtcgttgtaggtcagcaacagctggcgctgtgcctgccgcaccatgtcctcctggtcctcggtcaccatgtccagcaccttcaggaagtcctccactgccccatcgaactcctggagccgtcggtacatggtgccccggaagaggaagagactggggtccagagggttgttctcgatggcacggttgatccgctgcagtgcgtgctgcagcttgccctgcacagccaggatccccgcatcttggcgcgcctgctgggcctgggccaccatcttctggagcagcatcctggcctgcgggtgcttgggattcaacagcaaggcgctgtgcaggtcccggtagcagaggtggggcttctggagaaagttgtagagtctggcccggaagatgtagacatcggcgttggtggtgtcctgcttcagctcgttggtgatgagcgtgaggcaggcctgatgctgcttgagggccaggagacaggccatgcatcggtaacggaagcatggtttctcaggctggagctcagcagcatgtgagaagacattcagggcatccaggaaggcacactgctcaaaaaggcattgtccctgtaggtagagcacaaaggtgaggcgctccaggtgcttgcagttgtcctgctgtaatgagtaggcccttcgcaggttctgggcggccgaggagaagtcacagagctggaggtaggcctcagcccgtaaggcatagaagtccaccagctgtgggtccaggtggagtgcgcgggagaagagcagcacagctgtctcccagtctgcctgctccaagcactgctggcctctggagtagtattccctgactttgaggggcactgttaaccctgtgacctttggttttacatcacagatgctttggaacacgtggctggtcccaaagatgtgctgcaggatccctttgggggctggaatcacccatggctttgggatgtcccgtgaggggccctggtcaaccttcagggcatcctcgtccgaatctgtcatgaggccccttccaggaggaccccgaggcctctgccaactacctcgcggccctggccctgacgttgct

SEQ ID NO: 9678 - RNA, 1412 nt, Homo sapiens
  source 1..1412: mol_type = other RNA
atccttgctatctgggtgctaagcacctcctccaccgacatgcccgggaagaggttggtcatcagcagggacagctttggttgcttggggttgaggagcaggacagtggccacatcctggcgggccccaaaaatgttctgcagcagctgccggctcttggcccggtacaggtagtactgggccttctgggggttgtgccggatggccgtggagaagtggttctctgccttctggaactgcttgcgcctctgctcgcagaagcccatcttctcctgcagcaggcccatgcgcgtgttggcgccctcgtcctgagggctcagcgccagcgcctgctggtagtccgcctcggcaaaggccaggttgcccagctggaagaagcaatcgcctcggttgatgtagagtcctttctcctgctgctcgtcccggagggccttgttcagcagcagcacgccctcctggtaggcgccctgcctgtagcagtgcacggcaaagtcgttgtaggtcagcaacagctggcgctgtgcctgccgcaccatgtcctcctggtcctcggtcaccatgtccagcaccttcaggaagtcctccactgccccatcgaactccggaagaggaagagactggggtccagagggttgttctcgatggcacggttgatccgctgcagtgcgtgctgcagcttgccctgcacagccaggatccccgcatcttggcgcgcctgctgggcctgggccaccatcttctggagcagcatcctggcctgcgggtgcttgggattcaacagcaaggcgctgtgcaggtcccggtagcagaggtggggcttctggagaaagttgtagagtctggcccggaagatgtagacatcggcgttggtggtgtcctgcttcagctcgttggtgatgagcgtgaggcaggcctgatgctgcttgagggccaggagacaggccatgcatcggtaacggaagcatggtttctcaggctggagctcagcagcatgtgagaagacattcagggcatccaggaaggcacactgctcaaaaaggcattgtcccagctgtgggtccaggtggagtgcgcgggagaagagcagcacagctgtctcccagtctgcctgctccaagcactgctggcctctggagtagtattccctgactttgaggggcactgttaaccctgtgacctttggttttacatcacagatgctttggaacacgtggctggtcccaaagatgtgctgcaggatccctttgggggctggaatcacccatggctttgggatgtcccgtgaggggccctggtcaaccttcagggcatcctcgtccgaatctgtcatgaggccccttccaggaggaccccgaggcctctgccaactacctcgcggccctggccctgacgttgctaggcaccatcaccag

SEQ ID NO: 9679 - RNA, 1482 nt, Homo sapiens
  source 1..1482: mol_type = other RNA
atccttgctatctgggtgctaagcacctcctccaccgacatgcccgggaagaggttggtcatcagcagggacagctttggttgcttggggttgaggagcaggacagtggccacatcctggcgggccccaaaaatgttctgcagcagctgccggctcttggcccggtacaggtagtactgggccttctgggggttgtgccggatggccgtggagaagtggttctctgccttctggaactgcttgcgcctctgctcgcagaagcccatcttctcctgcagcaggcccatgcgcgtgttggcgccctcgtcctgagggctcagcgccagcgcctgctggtagtccgcctcggcaaaggccaggttgcccagctggaagaagcaatcgcctcggttgatgtagagtcctttctcctgctgctcgtcccggagggccttgttcagcagcagcacgccctcctggtaggcgccctgcctgtagcagtgcacggcaaagtcgttgtaggtcagcaacagctggcgctgtgcctgccgcaccatgtcctcctggtcctcggtcaccatgtccagcaccttcaggaagtcctccactgccccatcgaactccggaagaggaagagactggggtccagagggttgttctcgatggcacggttgatccgctgcagtgcgtgctgcagcttgccctgcacagccaggatccccgcatcttggcgcgcctgctgggcctgggccaccatcttctggagcagcatcctggcctgcgggtgcttgggattcaacagcaaggcgctgtgcaggtcccggtagcagaggtggggcttctggagaaagttgtagagtctggcccggaagatgtagacatcggcgttggtggtgtcctgcttcagctcgttggtgatgagcgtgaggcaggcctgatgctgcttgagggccaggagacaggccatgcatcggtaacggaagcatggtttctcaggctggagctcagcagcatgtgagaagacattcagggcatccaggaaggcacactgctcaaaaaggcattgtccctgtaggtagagcacaaaggtgaggcgctccaggtgcttgcagttgtcctgctgtaatgagtaggcccttcgcaggttctgggcggccgaggagaagtcacagagcagctgtgggtccaggtggagtgcgcgggagaagagcagcacagctgtctcccagtctgcctgctccaagcactgctggcctctggagtagtattccctgactttgaggggcactgttaaccctgtgacctttggttttacatcacagatgctttggaacacgtggctggtcccaaagatgtgctgcaggatccctttgggggctggaatcacccatggctttgggatgtcccgtgaggggccctggtcaaccttcagggcatcctcgtccgaatctgtcatgaggccccttccaggaggaccccgaggcctctgccaactacctcgcg

SEQ ID NO: 9680 - RNA, 1368 nt, Homo sapiens
  source 1..1368: mol_type = other RNA
atccttgctatctgggtgctaagcacctcctccaccgacatgcccgggaagaggttggtcatcagcagggacagctttggttgcttggggttgaggagcaggacagtggccacatcctggcgggccccaaaaatgttctgcagcagctgccggctcttggcccggtacaggtagtactgggccttctgggggttgtgccggatggccgtggagaagtggttctctgccttctggaactgcttgcgcctctgctcgcagaagcccatcttctcctgcagcaggcccatgcgcgtgttggcgccctcgtcctgagggctcagcgccagcgcctgctggtagtccgcctcggcaaaggccaggttgcccagctggaagaagcaatcgcctcggttgatgtagagtcctttctcctgctgctcgtcccggagggccttgttcagcagcagcacgccctcctggtaggcgccctgcctgtagcagtgcacggcaaagtcgttgtaggtcagcaacagctggcgctgtgcctgccgcaccatgtcctcctggtcctcggtcaccatgtccagcaccttcaggaagtcctccactgccccatcgaactccggaagaggaagagactggggtccagagggttgttctcgatggcacggttgatccgctgcagtgcgtgctgcagcttgccctgcacagccaggatccccgcatcttggcgcgcctgctgggcctgggccaccatcttctggagcagcatcctggcctgcgggtgcttgggattcaacagcaaggcgctgtgcaggtcccggtagcagaggtggggcttctggagaaagttgtagagtctggcccggaagatgtagacatcggcgttggtggtgtcctgcttcagctcgttggtgatgagcgtgaggcaggcctgatgctgcttgagggccaggagacaggccatgcatcggtaacggaagcatggtttctcaggctggagctcagcagcatgtgagaagacattcagggcatccaggaaggcacactgctcaaaaaggcattgtccctgtaggtagagcacaaaggtgaggcgctccaggtgcttgcagttgtcctgctgtaatgagtaggcccttcgcaggttctgggcggccgaggagaagtcacagagctggaggtaggcctcagcccgtaaggcatagaagtccaccagctgtgggtccaggtggagtgcgcgggagaagagcagcacagctgtctcccagtctgcctgctccaagcactgctggcctctggagtagctcgtccgaatctgtcatgaggccccttccaggaggaccccgaggcctctgccaactacctcgcggccctggccctgacgttgct

SEQ ID NO: 9681 - RNA, 1541 nt, Homo sapiens
  source 1..1541: mol_type = other RNA
atccttgctatctgggtgctaagcacctcctccaccgacatgcccgggaagaggttggtcatcagcagggacagctttggttgcttggggttgaggagcaggacagtggccacatcctggcgggccccaaaaatgttctgcagcagctgccggctcttggcccggtacaggtagtactgggccttctgggggttgtgccggatggccgtggagaagtggttctctgccttctggaactgcttgcgcctctgctcgcagaagcccatcttctcctgcagcaggcccatgcgcgtgttggcgccctcgtcctgagggctcagcgccagcgcctgctggtagtccgcctcggcaaaggccaggttgcccagctggaagaagcaatcgcctcggttgatgtagagtcctttctcctgctgctcgtcccggagggccttgttcagcagcagcacgccctcctggtaggcgccctgcctgtagcagtgcacggcaaagtcgttgtaggtcagcaacagctggcgctgtgcctgccgcaccatgtcctcctggtcctcggtcaccatgtccagcaccttcaggaagtcctccactgccccatcgaactccggaagaggaagagactggggtccagagggttgttctcgatggcacggttgatccgctgcagtgcgtgctgcagcttgccctgcacagccaggatccccgcatcttggcgcgcctgctgggcctgggccaccatcttctggagcagcatcctggcctgcgggtgcttgggattcaacagcaaggcgctgtgcaggtcccggtagcagaggtggggcttctggagaaagttgtagagtctggcccggaagatgtagacatcggcgttggtggtgtcctgcttcagctcgttggtgatgagcgtgaggcaggcctgatgctgcttgagggccaggagacaggccatgcatcggtaacggaagcatggtttctcaggctggagctcagcagcatgtgagaagacattcagggcatccaggaaggcacactgctcaaaaaggcattgtccctgtaggtagagcacaaaggtgaggcgctccaggtgcttgcagttgtcctgctgtaatgagtaggcccttcgcaggttctgggcggccgaggagaagtcacagagctggaggtaggcctcagcccgtaaggcatagaagtccaccagctgtgggtccaggtggagtgcgcgggagaagagcagcacagctgtctcccagtctgcctgctccaagcactgctggcctctggagtagtattccctgactttgaggggcactgttaaccctgtgacctttggttttacatcacagatgctttggaacacgtggctggtcccaaagatgtgctgcaggatccctttgggggctggaatcacccatggctttgggatgtcccgtgaggggccctggtcaaccttcagggcatcctcgtccgaatctgtcatgaggccccttccaggaggaccccgaggcctctgccaactacctcgcggccctggccctgacgttgct

SEQ ID NO: 9682 - RNA, 1437 nt, Homo sapiens
  source 1..1437: mol_type = other RNA
atccttgctatctgggtgctaagcacctcctccaccgacatgcccgggaagaggttggtcatcagcagggacagctttggttgcttggggttgaggagcaggacagtggccacatcctggcgggccccaaaaatgttctgcagcagctgccggctcttggcccggtacaggtagtactgggccttctgggggttgtgccggatggccgtggagaagtggttctctgccttctggaactgcttgcgcctctgctcgcagaagcccatcttctcctgcagcaggcccatgcgcgtgttggcgccctcgtcctgagggctcagcgccagcgcctgctggtagtccgcctcggcaaaggccaggttgcccagctggaagaagcaatcgcctcggttgatgtagagtcctttctcctgctgctcgtcccggagggccttgttcagcagcagcacgccctcctggtaggcgccctgcctgtagcagtgcacggcaaagtcgttgtaggtcagcaacagctggcgctgtgcctgccgcaccatgtcctcctggtcctcggtcaccatgtccagcaccttcaggaagtcctccactgccccatcgaactcctggagccgtcggtacatggtgccccggaagaggaagagactggggtccagagggttgttctcgatggcacggttgatccgctgcagtgcgtgctgcagcttgccctgcacagccaggatccccgcatcttggcgcgcctgctgggcctgggccaccatcttctggagcagcatcctggcctgcgggtgcttgggattcaacagcaaggcgctgtgcaggtcccggtagcagaggtggggcttctggagaaagttgtagagtctggcccggaagatgtagacatcggcgttggtggtgtcctgcttcagctcgttggtgatgagcgtgaggcaggcctgatgctgcttgagggccaggagacaggccatgcatcggtaacggaagcatggtttctcaggctggagctcagcagcatgtgagaagacattcagggcatccaggaaggcacactgctcaaaaaggcattgtcccagctgtgggtccaggtggagtgcgcgggagaagagcagcacagctgtctcccagtctgcctgctccaagcactgctggcctctggagtagtattccctgactttgaggggcactgttaaccctgtgacctttggttttacatcacagatgctttggaacacgtggctggtcccaaagatgtgctgcaggatccctttgggggctggaatcacccatggctttgggatgtcccgtgaggggccctggtcaaccttcagggcatcctcgtccgaatctgtcatgaggccccttccaggaggaccccgaggcctctgccaactacctcgcggccctggccctgacgttgctaggcaccatcaccag

SEQ ID NO: 9683 - RNA, 1527 nt, Homo sapiens
  source 1..1527: mol_type = other RNA
atccttgctatctgggtgctaagcacctcctccaccgacatgcccgggaagaggttggtcatcagcagggacagctttggttgcttggggttgaggagcaggacagtggccacatcctggcgggccccaaaaatgttctgcagcagctgccggctcttggcccggtacaggtagtactgggccttctgggggttgtgccggatggccgtggagaagtggttctctgccttctggaactgcttgcgcctctgctcgcagaagcccatcttctcctgcagcaggcccatgcgcgtgttggcgccctcgtcctgagggctcagcgccagcgcctgctggtagtccgcctcggcaaaggccaggttgcccagctggaagaagcaatcgcctcggttgatgtagagtcctttctcctgctgctcgtcccggagggccttgttcagcagcagcacgccctcctggtaggcgccctgcctgtagcagtgcacggcaaagtcgttgtaggtcagcaacagctggcgctgtgcctgccgcaccatgtcctcctggtcctcggtcaccatgtccagcaccttcaggaagtcctccactgccccatcgaactcctggagccgtcggtacatggtgccccggaagaggaagagactggggtccagagggttgttctcgatggcacggttgatccgctgcagtgcgtgctgcagcttgccctgcacagccaggatccccgcatcttggcgcgcctgctgggcctgggccaccatcttctggagcagcatcctggcctgcgggtgcttgggattcaacagcaaggcgctgtgcaggtcccggtagcagaggtggggcttctggagaaagttgtagagtctggcccggaagatgtagacatcggcgttggtggtgtcctgcttcagctcgttggtgatgagcgtgaggcaggcctgatgctgcttgagggccaggagacaggccatgcatcggtaacggaagcatggtttctcaggctggagctcagcagcatgtgagaagacattcagggcatccaggaaggcacactgctcaaaaaggcattgtccctgtaggtagagcacaaaggtgaggcgctccaggtgcttgcagttgtcctgctgtaatgagtaggcccttcgcaggttctgggcggccgaggagaagtcacagagcagctgtgggtccaggtggagtgcgcgggagaagagcagcacagctgtctcccagtctgcctgctccaagcactgctggcctctggagtagtattccctgactttgaggggcactgttaaccctgtgacctttggttttacatcacagatgctttggaacacgtggctggtcccaaagatgtgctgcaggatccctttgggggctggaatcacccatggctttgggatgtcccgtgaggggccctggtcaaccttcagggcatcctcgtccgaatctgtcatgaggccccttccaggaggaccccgaggcctctgccaactacctcgcggccctggccctgacgttgct

SEQ ID NO: 9684 - RNA, 1393 nt, Homo sapiens
  source 1..1393: mol_type = other RNA
atccttgctatctgggtgctaagcacctcctccaccgacatgcccgggaagaggttggtcatcagcagggacagctttggttgcttggggttgaggagcaggacagtggccacatcctggcgggccccaaaaatgttctgcagcagctgccggctcttggcccggtacaggtagtactgggccttctgggggttgtgccggatggccgtggagaagtggttctctgccttctggaactgcttgcgcctctgctcgcagaagcccatcttctcctgcagcaggcccatgcgcgtgttggcgccctcgtcctgagggctcagcgccagcgcctgctggtagtccgcctcggcaaaggccaggttgcccagctggaagaagcaatcgcctcggttgatgtagagtcctttctcctgctgctcgtcccggagggccttgttcagcagcagcacgccctcctggtaggcgccctgcctgtagcagtgcacggcaaagtcgttgtaggtcagcaacagctggcgctgtgcctgccgcaccatgtcctcctggtcctcggtcaccatgtccagcaccttcaggaagtcctccactgccccatcgaactcctggagccgtcggtacatggtgccccggaagaggaagagactggggtccagagggttgttctcgatggcacggttgatccgctgcagtgcgtgctgcagcttgccctgcacagccaggatccccgcatcttggcgcgcctgctgggcctgggccaccatcttctggagcagcatcctggcctgcgggtgcttgggattcaacagcaaggcgctgtgcaggtcccggtagcagaggtggggcttctggagaaagttgtagagtctggcccggaagatgtagacatcggcgttggtggtgtcctgcttcagctcgttggtgatgagcgtgaggcaggcctgatgctgcttgagggccaggagacaggccatgcatcggtaacggaagcatggtttctcaggctggagctcagcagcatgtgagaagacattcagggcatccaggaaggcacactgctcaaaaaggcattgtccctgtaggtagagcacaaaggtgaggcgctccaggtgcttgcagttgtcctgctgtaatgagtaggcccttcgcaggttctgggcggccgaggagaagtcacagagctggaggtaggcctcagcccgtaaggcatagaagtccaccagctgtgggtccaggtggagtgcgcgggagaagagcagcacagctgtctcccagtctgcctgctccaagcactgctggcctctggagtagctcgtccgaatctgtcatgaggccccttccaggaggaccccgaggcctctgccaactacctcgcggccctggccctgacgttgct

SEQ ID NO: 9685 - RNA, 1566 nt, Homo sapiens
  source 1..1566: mol_type = other RNA
atccttgctatctgggtgctaagcacctcctccaccgacatgcccgggaagaggttggtcatcagcagggacagctttggttgcttggggttgaggagcaggacagtggccacatcctggcgggccccaaaaatgttctgcagcagctgccggctcttggcccggtacaggtagtactgggccttctgggggttgtgccggatggccgtggagaagtggttctctgccttctggaactgcttgcgcctctgctcgcagaagcccatcttctcctgcagcaggcccatgcgcgtgttggcgccctcgtcctgagggctcagcgccagcgcctgctggtagtccgcctcggcaaaggccaggttgcccagctggaagaagcaatcgcctcggttgatgtagagtcctttctcctgctgctcgtcccggagggccttgttcagcagcagcacgccctcctggtaggcgccctgcctgtagcagtgcacggcaaagtcgttgtaggtcagcaacagctggcgctgtgcctgccgcaccatgtcctcctggtcctcggtcaccatgtccagcaccttcaggaagtcctccactgccccatcgaactcctggagccgtcggtacatggtgccccggaagaggaagagactggggtccagagggttgttctcgatggcacggttgatccgctgcagtgcgtgctgcagcttgccctgcacagccaggatccccgcatcttggcgcgcctgctgggcctgggccaccatcttctggagcagcatcctggcctgcgggtgcttgggattcaacagcaaggcgctgtgcaggtcccggtagcagaggtggggcttctggagaaagttgtagagtctggcccggaagatgtagacatcggcgttggtggtgtcctgcttcagctcgttggtgatgagcgtgaggcaggcctgatgctgcttgagggccaggagacaggccatgcatcggtaacggaagcatggtttctcaggctggagctcagcagcatgtgagaagacattcagggcatccaggaaggcacactgctcaaaaaggcattgtccctgtaggtagagcacaaaggtgaggcgctccaggtgcttgcagttgtcctgctgtaatgagtaggcccttcgcaggttctgggcggccgaggagaagtcacagagctggaggtaggcctcagcccgtaaggcatagaagtccaccagctgtgggtccaggtggagtgcgcgggagaagagcagcacagctgtctcccagtctgcctgctccaagcactgctggcctctggagtagtattccctgactttgaggggcactgttaaccctgtgacctttggttttacatcacagatgctttggaacacgtggctggtcccaaagatgtgctgcaggatccctttgggggctggaatcacccatggctttgggatgtcccgtgaggggccctggtcaaccttcagggcatcctcgtccgaatctgtcatgaggccccttccaggaggaccccgaggcctctgccaactacctcgcggccctggccctgacgttgct

SEQ ID NO: 9686 - RNA, 995 nt, Homo sapiens
  source 1..995: mol_type = other RNA
atcgctgcggttgcgagcgctgtagggagcctgtgctgtgccgcgcagttaggcagcagcagccgcggagcagtagccgccgtgggagggagccatgaagcattacgaggtaagaagcgagaaacaggggccgtgtggccactgctgacccattctttttccttctttgcgggaccacgggaccccactttctggtcctgtgccccgaaggaagagccagacggcgcaggcgcagtgggcaagcgttgcgccccgggccactcgtaaattccaatgcgcatgtgcgcaggaagtatttataaatctgcaacccaggctgttttgggggtactttttcttgggggtctctgcaggggctgggacgcttgcaggttccttgcagctcccccagcgggctgagttgcagactttgtcatgggagccacgaaggtgcgggacccttgctcccaatccgagggagtcttgcacaaatcttgcgccacgccgccgtcaccagcgtaggaaggggctttgctatcagtattcttgtgtacgacctttggaccccttccctcgcccgggacgttcccgggagacttaggcggtgagggaggtgcagctccacggctggctttcgcagagcagcgaagctgatcttgctttctggttatcaaagaggtcatctacgtcaacccttgggtgtcaccaaggagaaatcttatacccacccacagccactcttgaagcccaagtcttctgactcctaacttgggtctctttttcccttaaaacgaagtcttctgatgtgcttatcgccctaggtgataatataatattaataattcaaccaattatccctgaattattgctgacttttaagtaactatcatcaaataataaaatttgttattaaaattcaaaataacaatttagcaagtgcttactcttgtgctggtgagattctgttaccttgtataagaactattattattcctgtttgtaaggatgaataaagt

SEQ ID NO: 9687 - RNA, 70 nt, Homo sapiens
  source 1..70: mol_type = other RNA
atcgctttaccattcatgtttttaaaatctacctttcagtgaacatgaatggtaaagcgatgtcacattg

SEQ ID NO: 9688 - RNA, 65 nt, Homo sapiens
  source 1..65: mol_type = other RNA
atctaaatgcagcatgccagtccctgcatctcaggactggcatgctgcatttagatattagcagt

SEQ ID NO: 9689 - RNA, 443 nt, Homo sapiens
  source 1..443: mol_type = other RNA
atctgtaagagaaagtaaatgaaaaatctaagtcaatgagccgaagcagttttgtacttcgcatcctgaatggaaacagggatcgcctccatgtttcccttctttccaggacctcggctcttcagggcccagcggccttggttgctccggtatattcaatcagctggagtgtttttgttgttttaaatccaacttttacccttgttttagctggaggatttctctgatacaagccattccatcaagaaagtaggactctgtacatattcttttgtaagatgcttttctcgtatcactggagcgtttttcatgacattatatcctcagagtatccatcgttttgatacctatatttcatacctgatagaatgctgcctatgcagacattgtaccaatttgtttcaagcaagctttttctctacattctcatcagtactgaagta

SEQ ID NO: 9690 - RNA, 1600 nt, Homo sapiens
  source 1..1600: mol_type = other RNA
atctgtaagagaaagtaaatgaaaaatctaagtcaatgagccgaagcagttttgtacttcgcatcctgtcctgggctccttttcaaattctgttctacctcgcttctgaaacagtttcaaagataactcgccaatcctttcattttctgcattaatagctctttgaatttcttgtatttcctttttttgagctagaggaagttcttccagtttttctcttgactcaggttcattactgctttcatcatcatcaccatcacaaacctcaaagtcatcttcatagtcttcaaaatcatcttcacaactggctgtatatgcatcagctctagcattttctaaatcagtttcttccttttcaatttccacggtttcctcgcctcccggcctctggtccagcttccaccacacagaagagccttcctcgtggccatgcttccgtcttgaatctttatcttttccatgattccttactaaattctcagcatgctggctgctggtcccatctctttttgagcttgcacctcgatttctgtgttcaccattctgggattcccttttcctgggctcatcttttgccgatttctcttttctatccacgttgctttggtgcctctcatcatcaaaatgaaaaccttctttgtgtcgcttttctttatgtctttcttcccctttgtcagagaatgaattacttttctctttggaatatttctctcttttttcccttgtgctgcttttttctcggtgtttgttgtctcgatctggctctctgggcttcctgtgtctcctctcgccttcttctttataaagccagtacttgagagggttgtccttgctgtctccgtactgcagctttctttctcggtatcttctttctctatcttcatctcctctttcagagtcttcatctttctcttcacttcttactttacttactgagcggcctttcctctccgcccgctccaggagctgccggtcgcgtgtctcctggcccagcaggttgtggtgggccacggtctgccggagctcttccttccgggcccttctgtctttttctttttccctgtcctttcctctgctgtgagacttttctgcctctcgatgtttctccttcagcttttctttctcccggtcttttgcgtctcttctcctctccctctgtctgtctctgtccctctccccacgaggactctccttagcggtgtggacttcggccaccctgtctctgctcctggcatcctggtcgggatccctgcacctcggctccttatgttcaggaaggtccatctcagactccttacgcagcttcttctctctgtgctttctttcttccttggaaccacctgactgtatggcccagagatgttttctgaggtcatctgctttccaggtatcatctttggttcttctcttcccgggctccatcgcttcccgcaggcccgggcggccgcggtgtcctcggccccggccaggcgcggtccaccccgaagaggccacctgtgccccgcacccttcgggaggcgcgtcccagcgcctagcaaccgacaagcaggagcagcagagggcccagaagcactgcccagcgtgccctgcggcctctccc

SEQ ID NO: 9691 - RNA, 1821 nt, Homo sapiens
  source 1..1821: mol_type = other RNA
atctgtaagagaaagtaaatgaaaaatctaagtcaatgagccgaagcagttttgtacttcgcatcttttgcttaagggcctgagtccgactcttttgacggtgtgaagctgaggcaaaatccacaaaaattccacaaacagaggctctggaaggggaactgtttgtatctgtagtcccagctactcgggaggctgaagcagaagaatcgcttgaatccaggaaatgaaggttgcagtgagccgagatcatgccactgtactccagcacgggagacatagtgagactctgtcctgggctccttttcaaattctgttctacctcgcttctgaaacagtttcaaagataactcgccaatcctttcattttctgcattaatagctctttgaatttcttgtatttcctttttttgagctagaggaagttcttccagtttttctcttgactcaggttcattactgctttcatcatcatcaccatcacaaacctcaaagtcatcttcatagtcttcaaaatcatcttcacaactggctgtatatgcatcagctctagcattttctaaatcagtttcttccttttcaatttccacggtttcctcgcctcccggcctctggtccagcttccaccacacagaagagccttcctcgtggccatgcttccgtcttgaatctttatcttttccatgattccttactaaattctcagcatgctggctgctggtcccatctctttttgagcttgcacctcgatttctgtgttcaccattctgggattcccttttcctgggctcatcttttgccgatttctcttttctatccacgttgctttggtgcctctcatcatcaaaatgaaaaccttctttgtgtcgcttttctttatgtctttcttcccctttgtcagagaatgaattacttttctctttggaatatttctctcttttttcccttgtgctgcttttttctcggtgtttgttgtctcgatctggctctctgggcttcctgtgtctcctctcgccttcttctttataaagccagtacttgagagggttgtccttgctgtctccgtactgcagctttctttctcggtatcttctttctctatcttcatctcctctttcagagtcttcatctttctcttcacttcttactttacttactgagcggcctttcctctccgcccgctccaggagctgccggtcgcgtgtctcctggcccagcaggttgtggtgggccacggtctgccggagctcttccttccgggcccttctgtctttttctttttccctgtcctttcctctgctgtgagacttttctgcctctcgatgtttctccttcagcttttctttctcccggtcttttgcgtctcttctcctctccctctgtctgtctctgtccctctccccacgaggactctccttagcggtgtggacttcggccaccctgtctctgctcctggcatcctggtcgggatccctgcacctcggctccttatgttcaggaaggtccatctcagactccttacgcagcttcttctctctgtgctttctttcttccttggaaccacctgactgtatggcccagagatgttttctgaggtcatctgctttccaggtatcatctttggttcttctcttcccgggctccatcgcttcccgcaggcccgggcggccgcggtgtcctcggccccggccaggcgcggtccaccccgaagaggccacctgtgccccgcacccttcgggaggcgcgtcccagcgcctagcaaccgacaagcaggagcagcagagggcccagaagcactgcccagcgtgccctgcggcctctccc

SEQ ID NO: 9692 - RNA, 1940 nt, Homo sapiens
  source 1..1940: mol_type = other RNA
atctgtaagagaaagtaaatgaaaaatctaagtcaatgagccgaagcagttttgtacttcgcatcttttgcttaagggcctgagtccgactcttttgacggtgtgaagctgaggcaaaatccacaaaaattccacaaacagaggctctggaaggggaactgtttgtatctgtagtcccagctactcgggaggctgaagcagaagaatcgcttgaatccaggaaatgaaggttgcagtgagccgagatcatgccactgtactccagcacgggagacatagtgagactctgtcctgggctccttttcaaattctgttctacctcgcttctgaaacagtttcaaagataactcgccaatcctttcattttctgcattaatagctctttgaatttcttgtatttcctttttttgagctagaggaagttcttccagtttttctcttgactcaggttcattactgctttcatcatcatcaccatcacaaacctcaaagtcatcttcatagtcttcaaaatcatcttcacaactggctgtatatgcatcagctctagcattttctaaatcagtttcttccttttcaatttcctgtaaccccagctacttgggaggctgaagcaggagaatcacttgaacctgggaggcagaggttgcagcgagctgagatcgcaccattgcactccagcctgggcaatgacagcaaaactcacggtttcctcgcctcccggcctctggtccagcttccaccacacagaagagccttcctcgtggccatgcttccgtcttgaatctttatcttttccatgattccttactaaattctcagcatgctggctgctggtcccatctctttttgagcttgcacctcgatttctgtgttcaccattctgggattcccttttcctgggctcatcttttgccgatttctcttttctatccacgttgctttggtgcctctcatcatcaaaatgaaaaccttctttgtgtcgcttttctttatgtctttcttcccctttgtcagagaatgaattacttttctctttggaatatttctctcttttttcccttgtgctgcttttttctcggtgtttgttgtctcgatctggctctctgggcttcctgtgtctcctctcgccttcttctttataaagccagtacttgagagggttgtccttgctgtctccgtactgcagctttctttctcggtatcttctttctctatcttcatctcctctttcagagtcttcatctttctcttcacttcttactttacttactgagcggcctttcctctccgcccgctccaggagctgccggtcgcgtgtctcctggcccagcaggttgtggtgggccacggtctgccggagctcttccttccgggcccttctgtctttttctttttccctgtcctttcctctgctgtgagacttttctgcctctcgatgtttctccttcagcttttctttctcccggtcttttgcgtctcttctcctctccctctgtctgtctctgtccctctccccacgaggactctccttagcggtgtggacttcggccaccctgtctctgctcctggcatcctggtcgggatccctgcacctcggctccttatgttcaggaaggtccatctcagactccttacgcagcttcttctctctgtgctttctttcttccttggaaccacctgactgtatggcccagagatgttttctgaggtcatctgctttccaggtatcatctttggttcttctcttcccgggctccatcgcttcccgcaggcccgggcggccgcggtgtcctcggccccggccaggcgcggtccaccccgaagaggccacctgtgccccgcacccttcgggaggcgcgtcccagcgcctagcaaccgacaagcaggagcagcagagggcccagaagcactgcccagcgtgccctgcggcctctccc

SEQ ID NO: 9693 - RNA, 1647 nt, Homo sapiens
  source 1..1647: mol_type = other RNA
atctgtaagagaaagtaaatgaaaaatctaagtcaatgagccgaagcagttttgtacttcgcatcttttgcttaagggcctgagtccgactcttttgacggtgtgaagctgaggcaaaatccacaaaaattccacaaacagaggctctggaaggggaactgtttgtatctgtcctgggctccttttcaaattctgttctacctcgcttctgaaacagtttcaaagataactcgccaatcctttcattttctgcattaatagctctttgaatttcttgtatttcctttttttgagctagaggaagttcttccagtttttctcttgactcaggttcattactgctttcatcatcatcaccatcacaaacctcaaagtcatcttcatagtcttcaaaatcatcttcacaactggctgtatatgcatcagctctagcattttctaaatcagtttcttccttttcaatttccacggtttcctcgcctcccggcctctggtccagcttccaccacacagaagagccttcctcgtggccatgcttccgtcttgaatctttatcttttccatgattccttactaaattctcagcatgcctgggattcccttttcctgggctcatcttttgccgatttctcttttctatccacgttgctttggtgcctctcatcatcaaaatgaaaaccttctttgtgtcgcttttctttatgtctttcttcccctttgtcagagaatgaattacttttctctttggaatatttctctcttttttcccttgtgctgcttttttctcggtgtttgttgtctcgatctggctctctgggcttcctgtgtctcctctcgccttcttctttataaagccagtacttgagagggttgtccttgctgtctccgtactgcagctttctttctcggtatcttctttctctatcttcatctcctctttcagagtcttcatctttctcttcacttcttactttacttactgagcggcctttcctctccgcccgctccaggagctgccggtcgcgtgtctcctggcccagcaggttgtggtgggccacggtctgccggagctcttccttccgggcccttctgtctttttctttttccctgtcctttcctctgctgtgagacttttctgcctctcgatgtttctccttcagcttttctttctcccggtcttttgcgtctcttctcctctccctctgtctgtctctgtccctctccccacgaggactctccttagcggtgtggacttcggccaccctgtctctgctcctggcatcctggtcgggatccctgcacctcggctccttatgttcaggaaggtccatctcagactccttacgcagcttcttctctctgtgctttctttcttccttggaaccacctgactgtatggcccagagatgttttctgaggtcatctgctttccaggtatcatctttggttcttctcttcccgggctccatcgcttcccgcaggcccgggcggccgcggtgtcctcggccccggccaggcgcggtccaccccgaagaggccacctgtgccccgcacccttcgggaggcgcgtcccagcgcctagcaaccgacaagcaggagcagcagagggcccagaagcactgcccagcgtgccctgcggcctctccc

SEQ ID NO: 9694 - RNA, 1698 nt, Homo sapiens
  source 1..1698: mol_type = other RNA
atctgtaagagaaagtaaatgaaaaatctaagtcaatgagccgaagcagttttgtacttcgcatcttttgcttaagggcctgagtccgactcttttgacggtgtgaagctgaggcaaaatccacaaaaattccacaaacagaggctctggaaggggaactgtttgtatctgtcctgggctccttttcaaattctgttctacctcgcttctgaaacagtttcaaagataactcgccaatcctttcattttctgcattaatagctctttgaatttcttgtatttcctttttttgagctagaggaagttcttccagtttttctcttgactcaggttcattactgctttcatcatcatcaccatcacaaacctcaaagtcatcttcatagtcttcaaaatcatcttcacaactggctgtatatgcatcagctctagcattttctaaatcagtttcttccttttcaatttccacggtttcctcgcctcccggcctctggtccagcttccaccacacagaagagccttcctcgtggccatgcttccgtcttgaatctttatcttttccatgattccttactaaattctcagcatgctggctgctggtcccatctctttttgagcttgcacctcgatttctgtgttcaccattctgggattcccttttcctgggctcatcttttgccgatttctcttttctatccacgttgctttggtgcctctcatcatcaaaatgaaaaccttctttgtgtcgcttttctttatgtctttcttcccctttgtcagagaatgaattacttttctctttggaatatttctctcttttttcccttgtgctgcttttttctcggtgtttgttgtctcgatctggctctctgggcttcctgtgtctcctctcgccttcttctttataaagccagtacttgagagggttgtccttgctgtctccgtactgcagctttctttctcggtatcttctttctctatcttcatctcctctttcagagtcttcatctttctcttcacttcttactttacttactgagcggcctttcctctccgcccgctccaggagctgccggtcgcgtgtctcctggcccagcaggttgtggtgggccacggtctgccggagctcttccttccgggcccttctgtctttttctttttccctgtcctttcctctgctgtgagacttttctgcctctcgatgtttctccttcagcttttctttctcccggtcttttgcgtctcttctcctctccctctgtctgtctctgtccctctccccacgaggactctccttagcggtgtggacttcggccaccctgtctctgctcctggcatcctggtcgggatccctgcacctcggctccttatgttcaggaaggtccatctcagactccttacgcagcttcttctctctgtgctttctttcttccttggaaccacctgactgtatggcccagagatgttttctgaggtcatctgctttccaggtatcatctttggttcttctcttcccgggctccatcgcttcccgcaggcccgggcggccgcggtgtcctcggccccggccaggcgcggtccaccccgaagaggccacctgtgccccgcacccttcgggaggcgcgtcccagcgcctagcaaccgacaagcaggagcagcagagggcccagaagcactgcccagcgtgccctgcggcct

SEQ ID NO: 9695 - RNA, 1703 nt, Homo sapiens
  source 1..1703: mol_type = other RNA
atctgtaagagaaagtaaatgaaaaatctaagtcaatgagccgaagcagttttgtacttcgcatcttttgcttaagggcctgagtccgactcttttgacggtgtgaagctgaggcaaaatccacaaaaattccacaaacagaggctctggaaggggaactgtttgtatctgtcctgggctccttttcaaattctgttctacctcgcttctgaaacagtttcaaagataactcgccaatcctttcattttctgcattaatagctctttgaatttcttgtatttcctttttttgagctagaggaagttcttccagtttttctcttgactcaggttcattactgctttcatcatcatcaccatcacaaacctcaaagtcatcttcatagtcttcaaaatcatcttcacaactggctgtatatgcatcagctctagcattttctaaatcagtttcttccttttcaatttccacggtttcctcgcctcccggcctctggtccagcttccaccacacagaagagccttcctcgtggccatgcttccgtcttgaatctttatcttttccatgattccttactaaattctcagcatgctggctgctggtcccatctctttttgagcttgcacctcgatttctgtgttcaccattctgggattcccttttcctgggctcatcttttgccgatttctcttttctatccacgttgctttggtgcctctcatcatcaaaatgaaaaccttctttgtgtcgcttttctttatgtctttcttcccctttgtcagagaatgaattacttttctctttggaatatttctctcttttttcccttgtgctgcttttttctcggtgtttgttgtctcgatctggctctctgggcttcctgtgtctcctctcgccttcttctttataaagccagtacttgagagggttgtccttgctgtctccgtactgcagctttctttctcggtatcttctttctctatcttcatctcctctttcagagtcttcatctttctcttcacttcttactttacttactgagcggcctttcctctccgcccgctccaggagctgccggtcgcgtgtctcctggcccagcaggttgtggtgggccacggtctgccggagctcttccttccgggcccttctgtctttttctttttccctgtcctttcctctgctgtgagacttttctgcctctcgatgtttctccttcagcttttctttctcccggtcttttgcgtctcttctcctctccctctgtctgtctctgtccctctccccacgaggactctccttagcggtgtggacttcggccaccctgtctctgctcctggcatcctggtcgggatccctgcacctcggctccttatgttcaggaaggtccatctcagactccttacgcagcttcttctctctgtgctttctttcttccttggaaccacctgactgtatggcccagagatgttttctgaggtcatctgctttccaggtatcatctttggttcttctcttcccgggctccatcgcttcccgcaggcccgggcggccgcggtgtcctcggccccggccaggcgcggtccaccccgaagaggccacctgtgccccgcacccttcgggaggcgcgtcccagcgcctagcaaccgacaagcaggagcagcagagggcccagaagcactgcccagcgtgccctgcggcctctccc

SEQ ID NO: 9696 - RNA, 1764 nt, Homo sapiens
  source 1..1764: mol_type = other RNA
atctgtaagagaaagtaaatgaaaaatctaagtcaatgagccgaagcagttttgtacttcgcatcttttgcttaagggcctgagtccgactcttttgacggtgtgaagctgaggcaaaatccacaaaaattccacaaacagaggctctggaaggggaactgtttgtatctgtcctgggctccttttcaaattctgttctacctcgcttctgaaacagtttcaaagataactcgccaatcctttcattttctgcattaatagctctttgaatttcttgtatttcctttttttgagctagaggaagttcttccagtttttctcttgactcaggttcattactgctttcatcatcatcaccatcacaaacctcaaagtcatcttcatagtcttcaaaatcatcttcacaactggctgtatatgcatcagctctagcattttctaaatcagtttcttccttttcaatttccacggtttcctcgcctcccggcctctggtccagcttccaccacacagaagagccttcctcgtggccatgcttccgtcttgaatctttatcttttccatgattccttactaaattctcagcatgctggctgctggtcccatctctttttgagcttgcacctcgatttctgtgttcaccattctgggattcccttttcctgggctcatcttttgccgatttctcttttctatccacgttgctttggtgcctctcatcatcaaaatgaaaaccttctttgtgtcgcttttctttatgtctttcttcccctttgtcagagaatgaattacttttctctttggaatatttctctcttttttcccttgtgctgcttttttctcggtgtttgttgtctcgatctggctctctgggcttcctgtgtctcctctcgccttcttctttataaagccagtacttgagagggttgtccttgctgtctccgtactgcagctttctttctcggtatcttctttctctatcttcatctcctctttcagagtcttcatctttctcttcacttcttactttacttactgagcggcctttcctctccgcccgctccaggagctgccggtcgcgtgtctcctggcccagcaggttgtggtgggccacggtctgccggagctcttccttccgggcccttctgtctttttctttttccctgtcctttcctctgctgtgagacttttctgcctctcgatgtttctccttcagcttttctttctcccggtcttttgcgtctcttctcctctccctctgtctgtctctgtccctctccccacgaggactctccttagcggtgtggacttcggccaccctgtctctgctcctggcatcctggtcgggatccctgcacctcggctccttatgttcaggaaggtccatctcagactccttacgcagcttcttctctctgtgctttctttcttccttggaaccacctgactgtatggcccagagatgttttctgaggtcatctgctttccaggtatcatctttggttcttctcttcctttcccatcctctttaggttttgcagtcaggtgttacggagtcacattagcatcctctttaggttttgcagtcaggtgttacggagtcacattagcatcctctttaggttttgcagtcaggtgttacggagtcatattagcatcctctttaggttttgcagtcaggtgttacggagttacattagcatcctctttaggttttgcagtcagctgttatggagtcatattagcatcctctttaggttttgc

SEQ ID NO: 9697 - RNA, 1275 nt, Homo sapiens
  source 1..1275: mol_type = other RNA
atctgtaagagaaagtaaatgaaaaatctaagtcaatgagccgaagcagttttgtacttcgcatcttttgcttaagggcctgagtccgactcttttgacggtgtgaagctgaggcaaaatccacaaaaattccacaaacagaggctctggaaggggaactgtttgtatctgtcctgggctccttttcaaattctgttctacctcgcttctgaaacagtttcaaagataactcgccaatcctttcattttctgcattaatagctctttgaatttcttgtatttcctttttttgagctagaggaagttcttccagtttttctcttgactcaggttcattactgctttcatcatcatcaccatcacaaacctcaaagtcatcttcatagtcttcaaaatcatcttcacaactggctgtatatgcatcagctctagcattttctaaatcagtttcttccttttcaatttctctccttaccacggtttcctcgcctcccggcctctggtccagcttccaccacacagaagagccttcctcgtggccatgcttccgtcttgaatctttatcttttccatgattccttactaaattctcagcatgcctgggattcccttttcctgggctcatcttttgccgatttctcttttctatccacgttgctttggtgcctctcatcatcaaaatgaaaaccttctttgtgtcgcttttctttatgtctttcttcccctttgtcagagaatgaattacttttctctttggaatatttctctcttttttcccttgtgctgcttttttctcggtgtttgttgtctcgatctggctctctgggcttcctgtgtctcctctcgccttcttctttataaagccagtacttgagagggttgtccttgctgtctccgtactgcagctttctttctcggtatcttctttctctatcttcatctcctctttcagagtcttcatctttctcttcacttcttactttacttactgagcggcctttcctctccgcccgctccaggagctgccggtcgcgtgtctcctggcccagcaggttgtggtgggccacggtctgccggagctcttccttccgggcccttctgtctttttctttttccctgtcctttcctctgctgtgagacttttctgcctctcgatgtttctccttcagcttttctttctcccggtcttttgcgtctcttctcctctccctctgtctgtctctgtccctctccccacgaggactctccttagcggtgtggacttcggccaccctg

SEQ ID NO: 9698 - RNA, 1544 nt, Homo sapiens
  source 1..1544: mol_type = other RNA
atctgtaagagaaagtaaatgaaaaatctaagtcaatgagccgaagcagttttgtacttcgcatcttttgcttaagggcctgagtccgactcttttgacggtgtgaagctgaggcaaaatccacaaaaattccacaaacagaggctctggaaggggaactgtttgtatctgtcctgggctccttttcaaattctgttctacctcgcttctgaaacagtttcaaagataactcgccaatcctttcattttctgcattaatagctctttgaatttcttgtatttcctttttttgagctagaggaagttcttccagtttttctcttgactcaggttcattactgctttcatcatcatcaccatcacaaacctcaaagtcatcttcatagtcttcaaaatcatcttcacaactggctgtatatgcatcagctctagcattttctaaatcagtttcttccttttcaatttctctccttaccacggtttcctcgcctcccggcctctggtccagcttccaccacacagaagagccttcctcgtggccatgcttccgtcttgaatctttatcttttccatgattccttactaaattctcagcatgctggctgctggtcccatctctttttgagcttgcacctcgatttctgtgttcaccattctgggattcccttttcctgggctcatcttttgccgatttctcttttctatccacgttgctttggtgcctctcatcatcaaaatgaaaaccttctttgtgtcgcttttctttatgtctttcttcccctttgtcagagaatgaattacttttctctttggaatatttctctcttttttcccttgtgctgcttttttctcggtgtttgttgtctcgatctggctctctgggcttcctgtgtctcctctcgccttcttctttataaagccagtacttgagagggttgtccttgctgtctccgtactgcagctttctttctcggtatcttctttctctatcttcatctcctctttcagagtcttcatctttctcttcacttcttactttacttactgagcggcctttcctctccgcccgctccaggagctgccggtcgcgtgtctcctggcccagcaggttgtggtgggccacggtctgccggagctcttccttccgggcccttctgtctttttctttttccctgtcctttcctctgctgtgagacttttctgcctctcgatgtttctccttcagcttttctttctcccggtcttttgcgtctcttctcctctccctctgtctgtctctgtccctctccccacgaggactctccttagcggtgtggacttcggccaccctgtctctgctcctggcatcctggtcgggatccctgcacctcggctccttatgttcaggaaggtccatctcagactccttacgcagcttcttctctctgtgctttctttcttccttggaaccacctgactgtatggcccagagatgttttctgaggtcatctgctttccaggtatcatctttggttcttctctcttgactcagcatcaccaccaac

SEQ ID NO: 9699 - RNA, 1538 nt, Homo sapiens
  source 1..1538: mol_type = other RNA
atctgtaagagaaagtaaatgaaaaatctaagtcaatgagccgaagcagttttgtacttcgcatcttttgcttaagggcctgagtccgactcttttgacggtgtgaagctgaggcaaaatccacaaaaattccacaaacagaggctctggaaggggaactgtttgtatctgtcctgggctccttttcaaattctgttctacctcgcttctgaaacagtttcaaagataactcgccaatcctttcattttctgcattaatagctctttgaatttcttgtatttcctttttttgagctagaggaagttcttccagtttttctcttgactcaggttcattactgctttcatcatcatcaccatcacaaacctcaaagtcatcttcatagtcttcaaaatcatcttcacaactggctgtatatgcatcagctctagcattttctaaatcagtttcttccttttcaatttctctccttaccacggtttcctcgcctcccggcctctggtccagcttccaccacacagaagagccttcctcgtggccatgcttccgtcttgaatctttatcttttccatgattccttactaaattctcagcatgctggctgctggtcccatctctttttgagcttgcacctcgatttctgtgttcaccattctgggattcccttttcctgggctcatcttttgccgatttctcttttctatccacgttgctttggtgcctctcatcatcaaaatgaaaaccttctttgtgtcgcttttctttatgtctttcttcccctttgtcagagaatgaattacttttctctttggaatatttctctcttttttcccttgtgctgcttttttctcggtgtttgttgtctcgatctggctctctgggcttcctgtgtctcctctcgccttcttctttataaagccagtacttgagagggttgtccttgctgtctccgtactgcagctttctttctcggtatcttctttctctatcttcatctcctctttcagagtcttcatctttctcttcacttcttactttacttactgagcggcctttcctctccgcccgctccaggagctgccggtcgcgtgtctcctggcccagcaggttgtggtgggccacggtctgccggagctcttccttccgggcccttctgtctttttctttttccctgtcctttcctctgctgtgagacttttctgcctctcgatgtttctccttcagcttttctttctcccggtcttttgcgtctcttctcctctccctctgtctgtctctgtccctctccccacgaggactctccttagcggtgtggacttcggccaccctgtctctgctcctggcatcctggtcgggatccctgcacctcggctccttatgttcaggaaggtccatctcagactccttacgcagcttcttctctctgtgctttctttcttccttggaaccacctgactgtatggcccagagatgttttctgaggtcatctgctttccaggtatcatctttggttcttctctggagctaaggaagtccc

SEQ ID NO: 9700 - RNA, 1707 nt, Homo sapiens
  source 1..1707: mol_type = other RNA
atctgtaagagaaagtaaatgaaaaatctaagtcaatgagccgaagcagttttgtacttcgcatcttttgcttaagggcctgagtccgactcttttgacggtgtgaagctgaggcaaaatccacaaaaattccacaaacagaggctctggaaggggaactgtttgtatctgtcctgggctccttttcaaattctgttctacctcgcttctgaaacagtttcaaagataactcgccaatcctttcattttctgcattaatagctctttgaatttcttgtatttcctttttttgagctagaggaagttcttccagtttttctcttgactcaggttcattactgctttcatcatcatcaccatcacaaacctcaaagtcatcttcatagtcttcaaaatcatcttcacaactggctgtatatgcatcagctctagcattttctaaatcagtttcttccttttcaatttctctccttaccacggtttcctcgcctcccggcctctggtccagcttccaccacacagaagagccttcctcgtggccatgcttccgtcttgaatctttatcttttccatgattccttactaaattctcagcatgctggctgctggtcccatctctttttgagcttgcacctcgatttctgtgttcaccattctgggattcccttttcctgggctcatcttttgccgatttctcttttctatccacgttgctttggtgcctctcatcatcaaaatgaaaaccttctttgtgtcgcttttctttatgtctttcttcccctttgtcagagaatgaattacttttctctttggaatatttctctcttttttcccttgtgctgcttttttctcggtgtttgttgtctcgatctggctctctgggcttcctgtgtctcctctcgccttcttctttataaagccagtacttgagagggttgtccttgctgtctccgtactgcagctttctttctcggtatcttctttctctatcttcatctcctctttcagagtcttcatctttctcttcacttcttactttacttactgagcggcctttcctctccgcccgctccaggagctgccggtcgcgtgtctcctggcccagcaggttgtggtgggccacggtctgccggagctcttccttccgggcccttctgtctttttctttttccctgtcctttcctctgctgtgagacttttctgcctctcgatgtttctccttcagcttttctttctcccggtcttttgcgtctcttctcctctccctctgtctgtctctgtccctctccccacgaggactctccttagcggtgtggacttcggccaccctgtctctgctcctggcatcctggtcgggatccctgcacctcggctccttatgttcaggaaggtccatctcagactccttacgcagcttcttctctctgtgctttctttcttccttggaaccacctgactgtatggcccagagatgttttctgaggtcatctgctttccaggtatcatctttggttcttctcttcccgggctccatcgcttcccgcaggcccgggcggccgcggtgtcctcggccccggccaggcgcggtccaccccgaagaggccacctgtgccccgcacccttcgggaggcgcgtcccagcgcctagcaaccgacaagcaggagcagcagagggcccagaagcactgcccagcgtgccctgcggcct

SEQ ID NO: 9701 - RNA, 1728 nt, Homo sapiens
  source 1..1728: mol_type = other RNA
atctgtaagagaaagtaaatgaaaaatctaagtcaatgagccgaagcagttttgtacttcgcatcttttgcttaagggcctgagtccgactcttttgacggtgtgaagctgaggcaaaatccacaaaaattccacaaacagaggctctggaaggggaactgtttgtatctgtcctgggctccttttcaaattctgttctacctcgcttctgaaacagtttcaaagataactcgccaatcctttcattttctgcattaatagctctttgaatttcttgtatttcctttttttgagctagaggaagttcttccagtttttctcttgactcaggttcattactgctttcatcatcatcaccatcacaaacctcaaagtcatcttcatagtcttcaaaatcatcttcacaactggctgtatatgcatcagctctagcattttctaaatcagtttcttccttttcaatttctctccttaccacggtttcctcgcctcccggcctctggtccagcttccaccacacagaagagccttcctcgtggccatgcttccgtcttgaatctttatcttttccatgattccttactaaattctcagcatgctggctgctggtcccatctctttttgagcttgcacctcgatttctgtgttcaccattctgggattcccttttcctgggctcatcttttgccgatttctcttttctatccacgttgctttggtgcctctcatcatcaaaatgaaaaccttctttgtgtcgcttttctttatgtctttcttcccctttgtcagagaatgaattacttttctctttggaatatttctctcttttttcccttgtgctgcttttttctcggtgtttgttgtctcgatctggctctctgggcttcctgtgtctcctctcgccttcttctttataaagccagtacttgagagggttgtccttgctgtctccgtactgcagctttctttctcggtatcttctttctctatcttcatctcctctttcagagtcttcatctttctcttcacttcttactttacttactgagcggcctttcctctccgcccgctccaggagctgccggtcgcgtgtctcctggcccagcaggttgtggtgggccacggtctgccggagctcttccttccgggcccttctgtctttttctttttccctgtcctttcctctgctgtgagacttttctgcctctcgatgtttctccttcagcttttctttctcccggtcttttgcgtctcttctcctctccctctgtctgtctctgtccctctccccacgaggactctccttagcggtgtggacttcggccaccctgtctctgctcctggcatcctggtcgggatccctgcacctcggctccttatgttcaggaaggtccatctcagactccttacgcagcttcttctctctgtgctttctttcttccttggaaccacctgactgtatggcccagagatgttttctgaggtcatctgctttccaggtatcatctttggttcttctgtcccaaatgctgtgcacacagagggagtctgtgctccttctgcggccgctgggctcaacccaggacagaaggtatcatgggcctcccaggacaatgggtttctgcctggtcctcctgggctgcagctccagatacttccctgtgaggaagagaagcagccctggggagaggcccctgcagatgccacagcccagagggtccctcacag

SEQ ID NO: 9702 - RNA, 4909 nt, Homo sapiens
  source 1..4909: mol_type = other RNA
atctgtaagagaaagtaaatgaataacactcagtggccatggcgtgtttccccatctactagaacattctgtgacttacaccatctaccctgaaccattcaccacgtctccattcacgcagtgattcaaatagagttcctgtgttcattccacaataaacctcagtaattcgcacatcacagtacttgtaaccatttgttaacagaaagagaacgagtcttcatatatgagtttcttgtagacacagatagctgggtcttgattcgatccaacagcctctttcttttaatttgcatatgtacatcactgatgtttaattattgatatatgtggattaagagctacttactatatttgttactgttttccattctttctccatgtcttccattctttttcttctttctcttgtttcagttgagcactttatatgatttgttttttctcttttcaggggggcacaggttctatagtccaattattaggcctgagtcttataaggagtctctgggctgtgatcttcaaatgtgattctcagtccctggccctgcttagctggaatgggatagctatggggagctagatttgggtgtttcctttccctcagattaattaggttcttgtgaaacccagcaggttaggctctggttaggtagtttctcctgacagaaggccttgttaagaacagagtgttctggctgggtgtggtggctcacgcctgtaatcccagctacttgggaggctgaggcaggagaatcgcttgaacctgggaggcggagcttgcagtaagccgagatcgtgccattgcactccagcctgggtgacagagcaagactctgtctcaaaaaaaaagtgttctctcacatttttaaataattctctttttcttccccgcgccagaggtacaagggatttttctccaatatttactgtgagaatttcgtagagatctagcaggtaaagtgcacaaaagcatgtggacccccacatcaccaggccctctggagtcttcaattctcaggtttgtccatgttgagcctccaacaatctatcaatgacagtttaggtttccttgcactcacattggttcctgcggaggtttctactcatgggcttctgctccactatattcaatgcattcaacacgctagaacccttgcaggaaaccatgaacattgtctctacttggcagctgtggacacataaatccaaatcacacccctgcacctgccagaagcaaaggatgcccgtgatcaagggtttgaccccaagtcaaatgtcagtttctgaccccaaagccttcaggaacaaacaccctcgtctcctctgccttcattcctctcaagtctaacatgtctgtctcttccttattataataaaagtggaagcagattcaaggaaattaagttactcctaacacacagcttgaatccaatatttgattacagggtgtaccctgcattcttcatggcacttcatactacaaggatggcaaaacacaagactctgagcaggtcaaattccagtggcagaaacaagatgcatctccagaaaacagtaaagatgccataacggagacaaagacaataagcactgcgagaggtcagagggagaccagatgcccagagctccaaaaagctgacgataaccttcacagacaggtaggaggtgcatacccagaaaagacaggacatgttcgggcagttctactcactccaagttcagctcatcctaacaaagatgatgatatggtttggttgtgtccccacccaaatctcatcttgaattgcagctcccataattcccacaggtcatggtaggtatctggtgggaggtcattgaatgtctttcctgtgctattcttgtgacagtgaataaatcttacaagatctgatggttttataaaggtaagttcccctgcacatgctctcttgcctgctgccatgcaagacgtgactttgctcctcctttgccatccaccacgattgtgacgcctctccagccatgtggaaactctgagtcaattaaacctctttcctttgcaagttacccagtcttgggtaatgtctttattagcagcatgagaacagactaatacagacaacttgccaaattagacgggcaactcgcattcttctcaatccctccctgccggaggaacaagcatctcaactgagacgtgccccagtcaccacccatgttcccaagtcagcaccttgacctggtttccacatctccatcactagcacggaactcttgttggggtcataaagcttacttattttgcttttgtcttacttcttacctatgtttcagagttcagaaagaacatttaactaagatgaaaactgtattgtacagacactttgaccttgatgacatgagtcacattttacaacaaaatgcagatgccttataattctagtgcataagggcttccaagaccatcaagcagttctcaaacttcagtgtgcaaaagactgactgaggtgcttatttaaaatgcaaattttggggccccaacccagagattctgattcaaagggtactcaatatattatcttgttagaggttaatttaaaactttgaatattcaattgcaactctttacttcattttagagttttagcattgcacacatagcaaataaacatttattaattttatacttctctgcacatacagcaaatcaacatttattaattttatacttctttgccataaacagggtgtgcatccctggatagcagtgagcccttcagtgacctctgccctgggtcaaccgacattcgttcccattttaaagagggacagaggacagagaggaaagatcacctgcttcaggtgacacaccaggtaagaactggcatggaaactaacaactacgtctcttagatttcttacatcagaaatagatgtaacatcaaccagccctggttatctactctgtggagttcacactaaggaaaaagagacactgacttaaagtaaagacattttctttctctttcttttttttttaaaaaaaatattagtttaaagggaggggaggagtacaaatttaagatttccttgatcagaatttttttttttccacagtcggagttttgctccgtcacccaggctggagtgcagtggcgtgatctcggctcactgcagcctccaactcccaggttcaagcgattctcctgcctcagcctccagagtagctgggattacaggtgaacgccaccacgcctggctagtttttatattttttagtagagatggggttttaccatgttggccaagctggtcttgaactcctgaactcaagtgatccgcctgccactgcctcccaaagtgctgggattacaggcatgggccaccgtgcccagcctcttcgatcagattttaaacaactatatatttgtgaactcatttactcagggacacacagtgtttttattattattattgtttgtattttttgagatggagtctcgctctgtcacccaggccatagtgcactggcgacatctcagctcacttcaacctctgtctcctgggttcaagtgatcctcctaactcagcctcctgagtagctgggactacaggcacatgccaccacgcccggccaatttttgtatttttagtacagacggggtttcgccatgttggccaggctggtctcgaactcccaacctcaggtaatccacctgccttggccttccaaagtgctgggattacaggtatgtgccactgcatccagcccgcacagtgtttaaaatattcctctaaggaaacaattccagcctgggtctaggcagctttctagggttttgcttgggcaaacagtgttatttccaaagtgtcctgtaacctgctgagtttaggagaaggagtggaaattcagagctcccttgatccaggagccagaagattaatgtttcgggggtcagcagggggttgctgtgacgggtgtgagtggcaccacaccggacaaatgcccccatgttttggtcatcacacaaaccagttcttgtcaaattcctccccagaaagtttcctgtggctccaggccatggggctgggatggtgcagattttaaatcatggaaacttcaagaacatacctactcttcctctctcctctctgtccaaggagcccccatctgagtacagactgaccgtcacccacctacaataaactacatctctgagcaaaacaccagctgggctggcaggtcagaaggcagcttccccaggtcactacccgccaggaagcacccagcgacccacgcaccactcactttgtcgcccctccgctgccctcgtcgttgtcggaagatgacgatgtagaagagccagggaagtaggcggaatccacgtggttggggctgccgctctgggccgggttgatgggcaaggaccgctcatacagcggcgtgtgcttcccttcgtgaggaatgttgctgtagctgttctgctccgtcagattcttcccgctcgtgtccaaagtgagaggtgctggctcagagaggctgtacgggtatggaccctggcccggggcgccccctgggctgggcacctgtggggccacgggctttgcttgcagagaggtctgcggaatgttgagcatctgaggaggaacatgcggcggcaccatcccaggcattccaaacggaccgggtctggctgccacgtagtgtggtggctgcagtgaccgaggcttgctggtcccagaataatgtccgcttgctctgttacatcccagaactgattctcagggattgggatctggaagatgctcggcaggaggctgcggccgcagcggcgctgggctggagagaaggtggcggcgtgagggtccggcggcgctggagacccggcgggcagcggccaaagcagggtcgggctgagcccagcat

SEQ ID NO: 9703 - RNA, 2714 nt, Homo sapiens
  source 1..2714: mol_type = other RNA
atctgtaagagaaagtaaatgagaaacagacaaatgaagtggtagctggaggacgtgggaatcagtacaggttttcacgcctgtttcagaaatgggagattctacagcacgctcgacactaacacatcacatccataacatatcacatccaatagacaggacagccaaaaacacaaaacaaaaaaagaatcaaatacccacacccagacacaatactcaacaacacaaatacccgaccaaagtctttaagaaagcaaaagaggccgggcacagtggctcacacctgtaatcccagcactctaggaggccaaggtgggtggaccacttgaggtcaggagttcgagaccagcctggccaacatggcaaaacctcgtctctactgaaaatataaaaattagccaggcatggtggcacacgcctgtaatcccagcagtttgggaggctgaggcaggaggctcatttaaggtcaggagttcgagaccagcccgggcaacatggcaaaaccccgtctctactaaaaatacaaaaagttagccaggtgtggtggtgcacgcctgtagtccaagctactcgggaggctgaggcaggagagttacttgaacccagtaggtgaaggttacagtgagccgagatcacaccactgcactccagcctgagcaacacagggagacactctctcaaaaaaaaaaaaaaaaaaaaaaagatagtctccaaaacacaagaggtaaggtttaagtcccattggcttacgacaggaagatatgtgcacatctgcagagctggtaacagggaggcaggcattccctctgatggttgctgtttcttaatgaggcatgtgttgtggtaactaccacaagggggaattgatagataagacagaagttttgaaacagacatcccagagtagatctgctgggcagtgcttagtgtccatctgaggtttgtaatgataaacgtaaggtacaactggtggccaggctggctgttttctcacctaatgatggtgacttgggtttgggcacagaggtgaatgattgggtttacccagggttagggttttactagcggaacagaatggagggagacagaggggtgtagggtggactacggaattgatgctacacaagagggaagtgaaggcagaaggttactcatgagaatgtcagggctggttagaagaatgaagggtgagggtggaaaagcagcctctatttaaaaggttataagacaatcaatgtcctcagggaataatcaggtttcaaataaagtcaggagatggatggaccattcaaaacaaagttaaggatagagagatttgccagccaccttctggaagtgatagatggtgcagagtgggagagatgaggtcgtatgtggggatggacacagtagctggaggtgagcactcccgtacacagggtgactagaaaggcggggagaacagcacgaggcaccatgggctcctgagcgtctcttagaggcaggtgggtgttaggtcctagggctgtcatcctgaatgcttaaattggtatgaactgcaagcaggcaaggaagcaggagtgctcccagctgttaaacacatgcaagaaggcccagagcacggcctggcactttctaagtgcccaataagaaagaacaaaccacctgggaaagactccagccatttcccatttcctccccattcagcccacccacccacaaggtctctaataaatagggagcagtttttcacttcatcacaatctccctcccccgagagagccactcagacaccagaacaagtcaccaacccaccaggggtttaattctctgaatcaaaagatcagttcagagaggagccctgctttgtcctcatgcaggggtgaagatgtgcagagcaccctgggaatgtccaagcccagaagagccaggggccagtccctgagcaagtggagaattgggtcctggagtctcaggctgcctcctcctcttcactctcctcctcactctcatgatactgtctgcggtttgtgttaacaaacaggtcagaatcatcttctgagctggactcctctcctgataactgtggctcagctgggagttctggttgagtttgtctgttcctgttgttgtgtttctcagccacttcagagaaggcctcaggccaaaacccctccttctgcagagagcgcacgtggtccttgcagagcacaaacgagatttcagccttcaccttttctccctcttcaatggggtcaacaatgagaaagtcccctctcttgatccagatgttcttgcggtatttggagggcatgctcaccaggaagcgctgcccttgggctgtctccacctcatgcagattgttccctggggtcctgagtaccctgacaatctgctgctggtcggagggcactatgtgctcccctagcacctccttcaccacatgcttcctcttggtggcctgagacatgctgaagtcgtcccacaacttagtctctggccctcggctcccaggaacgctgccggagcaacaccgccgtctaggctggacgctgagagaggatcgtccacgactcacttcaaggctgaaccaagaaaacacagtaaaggaacttgccggcggccgcgacggtagcgtcagttagaaatcaggtctccagtgttcccagttcccaccagtccaactgcgaggagtgcgacgtgagtctgagtctgatccctccgaaaaccgtact

SEQ ID NO: 9704 - RNA, 2584 nt, Homo sapiens
  source 1..2584: mol_type = other RNA
atctgtaagagaaagtaaatgagaaacagacaaatgaagtggtagctggaggacgtgggaatcagtacaggttttcacgcctgtttcagaaatgggagattctacagcacgctcgacactaacacatcacatccataacatatcacatccaatagacaggacagccaaaaacacaaaacaaaaaaagaatcaaatacccacacccagacacaatactcaacaacacaaatacccgaccaaagtctttaagaaagcaaaagaggccgggcacagtggctcacacctgtaatcccagcactctaggaggccaaggtgggtggaccacttgaggtcaggagttcgagaccagcctggccaacatggcaaaacctcgtctctactgaaaatataaaaattagccaggcatggtggcacacgcctgtaatcccagcagtttgggaggctgaggcaggaggctcatttaaggtcaggagttcgagaccagcccgggcaacatggcaaaaccccgtctctactaaaaatacaaaaagttagccaggtgtggtggtgcacgcctgtagtccaagctactcgggaggctgaggcaggagagttacttgaacccagtaggtgaaggttacagtgagccgagatcacaccactgcactccagcctgagcaacacagggagacactctctcaaaaaaaaaaaaaaaaaaaaaaagatagtctccaaaacacaagaggtaaggtttaagtcccattggcttacgacaggaagatatgtgcacatctgcagagctggtaacagggaggcaggcattccctctgatggttgctgtttcttaatgaggcatgtgttgtggtaactaccacaagggggaattgatagataagacagaagttttgaaacagacatcccagagtagatctgctgggcagtgcttagtgtccatctgaggtttgtaatgataaacgtaaggtacaactggtggccaggctggctgttttctcacctaatgatggtgacttgggtttgggcacagaggtgaatgattgggtttacccagggttagggttttactagcggaacagaatggagggagacagaggggtgtagggtggactacggaattgatgctacacaagagggaagtgaaggcagaaggttactcatgagaatgtcagggctggttagaagaatgaagggtgagggtggaaaagcagcctctatttaaaaggttataagacaatcaatgtcctcagggaataatcaggtttcaaataaagtcaggagatggatggaccattcaaaacaaagttaaggatagagagatttgccagccaccttctggaagtgatagatggtgcagagtgggagagatgaggtcgtatgtggggatggacacagtagctggaggtgagcactcccgtacacagggtgactagaaaggcggggagaacagcacgaggcaccatgggctcctgagcgtctcttagaggcaggtgggtgttaggtcctagggctgtcatcctgaatgcttaaattggtatgaactgcaagcaggcaaggaagcaggagtgctcccagctgttaaacacatgcaagaaggcccagagcacggcctggcactttctaagtgcccaataagaaagaacaaaccacctgggaaagactccagccatttcccatttcctccccattcagcccacccacccacaaggtctctaataaatagggagcagtttttcacttcatcacaatctccctcccccgagagagccactcagacaccagaacaagtcaccaacccaccaggggtttaattctctgaatcaaaagatcagttcagagaggagccctgctttgtcctcatgcaggggtgaagatgtgcagagcaccctgggaatgtccaagcccagaagagccaggggccagtccctgagcaagtggagaattgggtcctggagtctcaggctgcctcctcctcttcactctcctcctcactctcatgatactgtctgcggtttgtgttaacaaacaggtcagaatcatcttctgagctggactcctctcctgataactgtggctcagctgggagttctggttgagtttgtctgttcctgttgttgtgtttctcagccacttcagagaaggcctcaggccaaaacccctccttctgcagagagcgcacgtggtccttgcagagcacaaacgagatttcagccttcaccttttctccctcttcaatggggtcaacaatgagaaagtcccctctcttgatccagatgttcttgcggtatttggagggcatgctcaccaggaagcgctgcccttgggctgtctccacctcatgcagattgttccctggggtcctgagtaccctgacaatctgctgctggtcggagggcactatgtgctcccctagcacctccttcaccacatgcttcctcttggtggcctgagacatgctgaagtcgtcccacacggcggccgcgacggtagcgtcagttagaaatcaggtctccagtgttcccagttcccaccagtccaactgcgaggagtgcgacgtgagtctgagtctgatccctccgaaaaccgtact

SEQ ID NO: 9705 - RNA, 2784 nt, Homo sapiens
  source 1..2784: mol_type = other RNA
atctgtaagagaaagtaaatgagaaacagacaaatgaagtggtagctggaggacgtgggaatcagtacaggttttcacgcctgtttcagaaatgggagattctacagcacgctcgacactaacacatcacatccataacatatcacatccaatagacaggacagccaaaaacacaaaacaaaaaaagaatcaaatacccacacccagacacaatactcaacaacacaaatacccgaccaaagtctttaagaaagcaaaagaggccgggcacagtggctcacacctgtaatcccagcactctaggaggccaaggtgggtggaccacttgaggtcaggagttcgagaccagcctggccaacatggcaaaacctcgtctctactgaaaatataaaaattagccaggcatggtggcacacgcctgtaatcccagcagtttgggaggctgaggcaggaggctcatttaaggtcaggagttcgagaccagcccgggcaacatggcaaaaccccgtctctactaaaaatacaaaaagttagccaggtgtggtggtgcacgcctgtagtccaagctactcgggaggctgaggcaggagagttacttgaacccagtaggtgaaggttacagtgagccgagatcacaccactgcactccagcctgagcaacacagggagacactctctcaaaaaaaaaaaaaaaaaaaaaaagatagtctccaaaacacaagaggtaaggtttaagtcccattggcttacgacaggaagatatgtgcacatctgcagagctggtaacagggaggcaggcattccctctgatggttgctgtttcttaatgaggcatgtgttgtggtaactaccacaagggggaattgatagataagacagaagttttgaaacagacatcccagagtagatctgctgggcagtgcttagtgtccatctgaggtttgtaatgataaacgtaaggtacaactggtggccaggctggctgttttctcacctaatgatggtgacttgggtttgggcacagaggtgaatgattgggtttacccagggttagggttttactagcggaacagaatggagggagacagaggggtgtagggtggactacggaattgatgctacacaagagggaagtgaaggcagaaggttactcatgagaatgtcagggctggttagaagaatgaagggtgagggtggaaaagcagcctctatttaaaaggttataagacaatcaatgtcctcagggaataatcaggtttcaaataaagtcaggagatggatggaccattcaaaacaaagttaaggatagagagatttgccagccaccttctggaagtgatagatggtgcagagtgggagagatgaggtcgtatgtggggatggacacagtagctggaggtgagcactcccgtacacagggtgactagaaaggcggggagaacagcacgaggcaccatgggctcctgagcgtctcttagaggcaggtgggtgttaggtcctagggctgtcatcctgaatgcttaaattggtatgaactgcaagcaggcaaggaagcaggagtgctcccagctgttaaacacatgcaagaaggcccagagcacggcctggcactttctaagtgcccaataagaaagaacaaaccacctgggaaagactccagccatttcccatttcctccccattcagcccacccacccacaaggtctctaataaatagggagcagtttttcacttcatcacaatctccctcccccgagagagccactcagacaccagaacaagtcaccaacccaccaggggtttaattctctgaatcaaaagatcagttcagagaggagccctgctttgtcctcatgcaggggtgaagatgtgcagagcaccctgggaatgtccaagcccagaagagccaggggccagtccctgagcaagtggagaattgggtcctggagtctcaggctgcctcctcctcttcactctcctcctcactctcatgatactgtctgcggtttgtgttaacaaacaggtcagaatcatcttctgagctggactcctctcctgataactgtggctcagctgggagttctggttgagtttgtctgttcctgttgttgtgtttctcagccacttcagagaaggcctcaggccaaaacccctccttctgcagagagcgcacgtggtccttgcagagcacaaacgagatttcagccttcaccttttctccctcttcaatggggtcaacaatgagaaagtcccctctcttgatccagatgttcttgcggtatttggagggcatgctcaccaggaagcgctgcccttgggctgtctccacctcatgcagattgttccctggggtcctgagtaccctgacaatctgctgctggtcggagggcactatgtgctcccctagcacctccttcaccacatgcttcctcttggtggcctgagacatgctgaagtcgtcccacactggttaggaacgaagagactgtcaactcctcctcctgagttccttggatggcaggctcagaacccaggaacttagtctctggccctcggctcccaggaacgctgccggagcaacaccgccgtctaggctggacgctgagagaggatcgtccacgactcacttcaaggctgaaccaagaaaacacagtaaaggaacttgccggcggccgcgacggtagcgtcagttagaaatcaggtctccagtgttcccagttcccaccagtccaactgcgaggagtgcgacgtgagtctgagtctgatccctccgaaaaccgtact

SEQ ID NO: 9706 - RNA, 2789 nt, Homo sapiens
  source 1..2789: mol_type = other RNA
atctgtaagagaaagtaaatgagaaacagacaaatgaagtggtagctggaggacgtgggaatcagtacaggttttcacgcctgtttcagaaatgggagattctacagcacgctcgacactaacacatcacatccataacatatcacatccaatagacaggacagccaaaaacacaaaacaaaaaaagaatcaaatacccacacccagacacaatactcaacaacacaaatacccgaccaaagtctttaagaaagcaaaagaggccgggcacagtggctcacacctgtaatcccagcactctaggaggccaaggtgggtggaccacttgaggtcaggagttcgagaccagcctggccaacatggcaaaacctcgtctctactgaaaatataaaaattagccaggcatggtggcacacgcctgtaatcccagcagtttgggaggctgaggcaggaggctcatttaaggtcaggagttcgagaccagcccgggcaacatggcaaaaccccgtctctactaaaaatacaaaaagttagccaggtgtggtggtgcacgcctgtagtccaagctactcgggaggctgaggcaggagagttacttgaacccagtaggtgaaggttacagtgagccgagatcacaccactgcactccagcctgagcaacacagggagacactctctcaaaaaaaaaaaaaaaaaaaaaaagatagtctccaaaacacaagaggtaaggtttaagtcccattggcttacgacaggaagatatgtgcacatctgcagagctggtaacagggaggcaggcattccctctgatggttgctgtttcttaatgaggcatgtgttgtggtaactaccacaagggggaattgatagataagacagaagttttgaaacagacatcccagagtagatctgctgggcagtgcttagtgtccatctgaggtttgtaatgataaacgtaaggtacaactggtggccaggctggctgttttctcacctaatgatggtgacttgggtttgggcacagaggtgaatgattgggtttacccagggttagggttttactagcggaacagaatggagggagacagaggggtgtagggtggactacggaattgatgctacacaagagggaagtgaaggcagaaggttactcatgagaatgtcagggctggttagaagaatgaagggtgagggtggaaaagcagcctctatttaaaaggttataagacaatcaatgtcctcagggaataatcaggtttcaaataaagtcaggagatggatggaccattcaaaacaaagttaaggatagagagatttgccagccaccttctggaagtgatagatggtgcagagtgggagagatgaggtcgtatgtggggatggacacagtagctggaggtgagcactcccgtacacagggtgactagaaaggcggggagaacagcacgaggcaccatgggctcctgagcgtctcttagaggcaggtgggtgttaggtcctagggctgtcatcctgaatgcttaaattggtatgaactgcaagcaggcaaggaagcaggagtgctcccagctgttaaacacatgcaagaaggcccagagcacggcctggcactttctaagtgcccaataagaaagaacaaaccacctgggaaagactccagccatttcccatttcctccccattcagcccacccacccacaaggtctctaataaatagggagcagtttttcacttcatcacaatctccctcccccgagagagccactcagacaccagaacaagtcaccaacccaccaggggtttaattctctgaatcaaaagatcagttcagagaggagccctgctttgtcctcatgcaggggtgaagatgtgcagagcaccctgggaatgtccaagcccagaagagccaggggccagtccctgagcaagtggagaattgggtcctggagtctcaggctgcctcctcctcttcactctcctcctcactctcatgatactgtctgcggtttgtgttaacaaacaggtcagaatcatcttctgagctggactcctctcctgataactgtggctcagctgggagttctggttgagtttgtctgttcctgttgttgtgtttctcagccacttcagagaaggcctcaggccaaaacccctccttctgcagagagcgcacgtggtccttgcagagcacaaacgagatttcagccttcaccttttctccctcttcaatggggtcaacaatgagaaagtcccctctcttgatccagatgttcttgcggtatttggagggcatgctcaccaggaagcgctgcccttgggctgtctccacctcatgcagattgttccctggggtcctgagtaccctgacaatctgctgctggtcggagggcactatgtgctcccctagcacctccttcaccacatgcttcctcttggtggcctgagacatgctgaagtcgtcccacactggttaggaacgaagagactgtcaactcctcctcctgagttccttggatggcaggctcagaacccaggactgttacttagtctctggccctcggctcccaggaacgctgccggagcaacaccgccgtctaggctggacgctgagagaggatcgtccacgactcacttcaaggctgaaccaagaaaacacagtaaaggaacttgccggcggccgcgacggtagcgtcagttagaaatcaggtctccagtgttcccagttcccaccagtccaactgcgaggagtgcgacgtgagtctgagtctgatccctccgaaaaccgtact

SEQ ID NO: 9707 - RNA, 2659 nt, Homo sapiens
  source 1..2659: mol_type = other RNA
atctgtaagagaaagtaaatgagaaacagacaaatgaagtggtagctggaggacgtgggaatcagtacaggttttcacgcctgtttcagaaatgggagattctacagcacgctcgacactaacacatcacatccataacatatcacatccaatagacaggacagccaaaaacacaaaacaaaaaaagaatcaaatacccacacccagacacaatactcaacaacacaaatacccgaccaaagtctttaagaaagcaaaagaggccgggcacagtggctcacacctgtaatcccagcactctaggaggccaaggtgggtggaccacttgaggtcaggagttcgagaccagcctggccaacatggcaaaacctcgtctctactgaaaatataaaaattagccaggcatggtggcacacgcctgtaatcccagcagtttgggaggctgaggcaggaggctcatttaaggtcaggagttcgagaccagcccgggcaacatggcaaaaccccgtctctactaaaaatacaaaaagttagccaggtgtggtggtgcacgcctgtagtccaagctactcgggaggctgaggcaggagagttacttgaacccagtaggtgaaggttacagtgagccgagatcacaccactgcactccagcctgagcaacacagggagacactctctcaaaaaaaaaaaaaaaaaaaaaaagatagtctccaaaacacaagaggtaaggtttaagtcccattggcttacgacaggaagatatgtgcacatctgcagagctggtaacagggaggcaggcattccctctgatggttgctgtttcttaatgaggcatgtgttgtggtaactaccacaagggggaattgatagataagacagaagttttgaaacagacatcccagagtagatctgctgggcagtgcttagtgtccatctgaggtttgtaatgataaacgtaaggtacaactggtggccaggctggctgttttctcacctaatgatggtgacttgggtttgggcacagaggtgaatgattgggtttacccagggttagggttttactagcggaacagaatggagggagacagaggggtgtagggtggactacggaattgatgctacacaagagggaagtgaaggcagaaggttactcatgagaatgtcagggctggttagaagaatgaagggtgagggtggaaaagcagcctctatttaaaaggttataagacaatcaatgtcctcagggaataatcaggtttcaaataaagtcaggagatggatggaccattcaaaacaaagttaaggatagagagatttgccagccaccttctggaagtgatagatggtgcagagtgggagagatgaggtcgtatgtggggatggacacagtagctggaggtgagcactcccgtacacagggtgactagaaaggcggggagaacagcacgaggcaccatgggctcctgagcgtctcttagaggcaggtgggtgttaggtcctagggctgtcatcctgaatgcttaaattggtatgaactgcaagcaggcaaggaagcaggagtgctcccagctgttaaacacatgcaagaaggcccagagcacggcctggcactttctaagtgcccaataagaaagaacaaaccacctgggaaagactccagccatttcccatttcctccccattcagcccacccacccacaaggtctctaataaatagggagcagtttttcacttcatcacaatctccctcccccgagagagccactcagacaccagaacaagtcaccaacccaccaggggtttaattctctgaatcaaaagatcagttcagagaggagccctgctttgtcctcatgcaggggtgaagatgtgcagagcaccctgggaatgtccaagcccagaagagccaggggccagtccctgagcaagtggagaattgggtcctggagtctcaggctgcctcctcctcttcactctcctcctcactctcatgatactgtctgcggtttgtgttaacaaacaggtcagaatcatcttctgagctggactcctctcctgataactgtggctcagctgggagttctggttgagtttgtctgttcctgttgttgtgtttctcagccacttcagagaaggcctcaggccaaaacccctccttctgcagagagcgcacgtggtccttgcagagcacaaacgagatttcagccttcaccttttctccctcttcaatggggtcaacaatgagaaagtcccctctcttgatccagatgttcttgcggtatttggagggcatgctcaccaggaagcgctgcccttgggctgtctccacctcatgcagattgttccctggggtcctgagtaccctgacaatctgctgctggtcggagggcactatgtgctcccctagcacctccttcaccacatgcttcctcttggtggcctgagacatgctgaagtcgtcccacactggttaggaacgaagagactgtcaactcctcctcctgagttccttggatggcaggctcagaacccaggactgttcggcggccgcgacggtagcgtcagttagaaatcaggtctccagtgttcccagttcccaccagtccaactgcgaggagtgcgacgtgagtctgagtctgatccctccgaaaaccgtact

SEQ ID NO: 9708 - RNA, 2813 nt, Homo sapiens
  source 1..2813: mol_type = other RNA
atctgtaagagaaagtaaatgagaaacagacaaatgaagtggtagctggaggacgtgggaatcagtacaggttttcacgcctgtttcagaaatgggagattctacagcacgctcgacactaacacatcacatccataacatatcacatccaatagacaggacagccaaaaacacaaaacaaaaaaagaatcaaatacccacacccagacacaatactcaacaacacaaatacccgaccaaagtctttaagaaagcaaaagaggccgggcacagtggctcacacctgtaatcccagcactctaggaggccaaggtgggtggaccacttgaggtcaggagttcgagaccagcctggccaacatggcaaaacctcgtctctactgaaaatataaaaattagccaggcatggtggcacacgcctgtaatcccagcagtttgggaggctgaggcaggaggctcatttaaggtcaggagttcgagaccagcccgggcaacatggcaaaaccccgtctctactaaaaatacaaaaagttagccaggtgtggtggtgcacgcctgtagtccaagctactcgggaggctgaggcaggagagttacttgaacccagtaggtgaaggttacagtgagccgagatcacaccactgcactccagcctgagcaacacagggagacactctctcaaaaaaaaaaaaaaaaaaaaaaagatagtctccaaaacacaagaggtaaggtttaagtcccattggcttacgacaggaagatatgtgcacatctgcagagctggtaacagggaggcaggcattccctctgatggttgctgtttcttaatgaggcatgtgttgtggtaactaccacaagggggaattgatagataagacagaagttttgaaacagacatcccagagtagatctgctgggcagtgcttagtgtccatctgaggtttgtaatgataaacgtaaggtacaactggtggccaggctggctgttttctcacctaatgatggtgacttgggtttgggcacagaggtgaatgattgggtttacccagggttagggttttactagcggaacagaatggagggagacagaggggtgtagggtggactacggaattgatgctacacaagagggaagtgaaggcagaaggttactcatgagaatgtcagggctggttagaagaatgaagggtgagggtggaaaagcagcctctatttaaaaggttataagacaatcaatgtcctcagggaataatcaggtttcaaataaagtcaggagatggatggaccattcaaaacaaagttaaggatagagagatttgccagccaccttctggaagtgatagatggtgcagagtgggagagatgaggtcgtatgtggggatggacacagtagctggaggtgagcactcccgtacacagggtgactagaaaggcggggagaacagcacgaggcaccatgggctcctgagcgtctcttagaggcaggtgggtgttaggtcctagggctgtcatcctgaatgcttaaattggtatgaactgcaagcaggcaaggaagcaggagtgctcccagctgttaaacacatgcaagaaggcccagagcacggcctggcactttctaagtgcccaataagaaagaacaaaccacctgggaaagactccagccatttcccatttcctccccattcagcccacccacccacaaggtctctaataaatagggagcagtttttcacttcatcacaatctccctcccccgagagagccactcagacaccagaacaagtcaccaacccaccaggggtttaattctctgaatcaaaagatcagttcagagaggagccctgctttgtcctcatgcaggggtgaagatgtgcagagcaccctgggaatgtccaagcccagaagagccaggggccagtccctgagcaagtggagaattgggtcctggagtctcaggctgcctcctcctcttcactctcctcctcactctcatgatactgtctgcggtttgtgttaacaaacaggtcagaatcatcttctgagctggactcctctcctgataactgtggctcagctgggagttctggttgagtttgtctgttcctgttgttgtgtttctcagccacttcagagaaggcctcaggccaaaacccctccttctgcagagagcgcacgtggtccttgcagagcacaaacgagatttcagccttcaccttttctccctcttcaatggggtcaacaatgagaaagtcccctctcttgatccagatgttcttgcggtatttggagggcatgctcaccaggaagcgctgcccttgggctgtctccacctcatgcagattgttccctggggtcctgagtaccctgacaatctgctgctggtcggagggcactatgtgctcccctagcacctccttcaccacatgcttcctcttggtggcctgagacatgctgaagtcgtcccacactggttaggaacgaagagactgtcaactcctcctcctgagttccttggatggcaggctcagaacccaggactgttctgaagatggggaggggccttttaacttagtctctggccctcggctcccaggaacgctgccggagcaacaccgccgtctaggctggacgctgagagaggatcgtccacgactcacttcaaggctgaaccaagaaaacacagtaaaggaacttgccggcggccgcgacggtagcgtcagttagaaatcaggtctccagtgttcccagttcccaccagtccaactgcgaggagtgcgacgtgagtctgagtctgatccctccgaaaaccgtact

SEQ ID NO: 9709 - RNA, 2683 nt, Homo sapiens
  source 1..2683: mol_type = other RNA
atctgtaagagaaagtaaatgagaaacagacaaatgaagtggtagctggaggacgtgggaatcagtacaggttttcacgcctgtttcagaaatgggagattctacagcacgctcgacactaacacatcacatccataacatatcacatccaatagacaggacagccaaaaacacaaaacaaaaaaagaatcaaatacccacacccagacacaatactcaacaacacaaatacccgaccaaagtctttaagaaagcaaaagaggccgggcacagtggctcacacctgtaatcccagcactctaggaggccaaggtgggtggaccacttgaggtcaggagttcgagaccagcctggccaacatggcaaaacctcgtctctactgaaaatataaaaattagccaggcatggtggcacacgcctgtaatcccagcagtttgggaggctgaggcaggaggctcatttaaggtcaggagttcgagaccagcccgggcaacatggcaaaaccccgtctctactaaaaatacaaaaagttagccaggtgtggtggtgcacgcctgtagtccaagctactcgggaggctgaggcaggagagttacttgaacccagtaggtgaaggttacagtgagccgagatcacaccactgcactccagcctgagcaacacagggagacactctctcaaaaaaaaaaaaaaaaaaaaaaagatagtctccaaaacacaagaggtaaggtttaagtcccattggcttacgacaggaagatatgtgcacatctgcagagctggtaacagggaggcaggcattccctctgatggttgctgtttcttaatgaggcatgtgttgtggtaactaccacaagggggaattgatagataagacagaagttttgaaacagacatcccagagtagatctgctgggcagtgcttagtgtccatctgaggtttgtaatgataaacgtaaggtacaactggtggccaggctggctgttttctcacctaatgatggtgacttgggtttgggcacagaggtgaatgattgggtttacccagggttagggttttactagcggaacagaatggagggagacagaggggtgtagggtggactacggaattgatgctacacaagagggaagtgaaggcagaaggttactcatgagaatgtcagggctggttagaagaatgaagggtgagggtggaaaagcagcctctatttaaaaggttataagacaatcaatgtcctcagggaataatcaggtttcaaataaagtcaggagatggatggaccattcaaaacaaagttaaggatagagagatttgccagccaccttctggaagtgatagatggtgcagagtgggagagatgaggtcgtatgtggggatggacacagtagctggaggtgagcactcccgtacacagggtgactagaaaggcggggagaacagcacgaggcaccatgggctcctgagcgtctcttagaggcaggtgggtgttaggtcctagggctgtcatcctgaatgcttaaattggtatgaactgcaagcaggcaaggaagcaggagtgctcccagctgttaaacacatgcaagaaggcccagagcacggcctggcactttctaagtgcccaataagaaagaacaaaccacctgggaaagactccagccatttcccatttcctccccattcagcccacccacccacaaggtctctaataaatagggagcagtttttcacttcatcacaatctccctcccccgagagagccactcagacaccagaacaagtcaccaacccaccaggggtttaattctctgaatcaaaagatcagttcagagaggagccctgctttgtcctcatgcaggggtgaagatgtgcagagcaccctgggaatgtccaagcccagaagagccaggggccagtccctgagcaagtggagaattgggtcctggagtctcaggctgcctcctcctcttcactctcctcctcactctcatgatactgtctgcggtttgtgttaacaaacaggtcagaatcatcttctgagctggactcctctcctgataactgtggctcagctgggagttctggttgagtttgtctgttcctgttgttgtgtttctcagccacttcagagaaggcctcaggccaaaacccctccttctgcagagagcgcacgtggtccttgcagagcacaaacgagatttcagccttcaccttttctccctcttcaatggggtcaacaatgagaaagtcccctctcttgatccagatgttcttgcggtatttggagggcatgctcaccaggaagcgctgcccttgggctgtctccacctcatgcagattgttccctggggtcctgagtaccctgacaatctgctgctggtcggagggcactatgtgctcccctagcacctccttcaccacatgcttcctcttggtggcctgagacatgctgaagtcgtcccacactggttaggaacgaagagactgtcaactcctcctcctgagttccttggatggcaggctcagaacccaggactgttctgaagatggggaggggccttttacggcggccgcgacggtagcgtcagttagaaatcaggtctccagtgttcccagttcccaccagtccaactgcgaggagtgcgacgtgagtctgagtctgatccctccgaaaaccgtact

SEQ ID NO: 9710 - RNA, 6288 nt, Homo sapiens
  source 1..6288: mol_type = other RNA
atgcacctgggcaaggattctgatagagaagaattttggctcatctctgaaaaaacattttcacatagaaattccttctctgggtttggcaaagcattctgatgacctttttgtaatgttggcacagaattttgttcttcactgattggcactacactatgattagtctggcaaattggctgattgggcagatcttgggtcactagtatttgtggcagggatgtgagtgtagcaaaacagtaagcaggaacactactctgcaggcgtatgggcagcatgaatgatgatggcaccttctgcacctgacttccaaggggcctgagctctggtggtagcagaggatgcgaattagacatgctgtcaattaatttggttggtaatgttgctgatgtcacacaatgatctgttccaactggatctgaaataacttgatttggcaaagaatgcacaggattagaagagcaagatgggcctgaagtgaaaacctgacaatgcaattggtatttgggagcaaagcaatcctcacttttagaagacccagataaaacagaatttttatctggcttgctaccctgcgtagacacttgcagagatagctgtgtgctctggtggctaggcggtgcatggatttgatttaacaaattgatatcacagagctgttgaacaggaaaaacgttggtagagctggagtttgatgtttctgcctgcagatccttaacctgagtctgagagtgcaaagtatttgcagaaaactcagctaaagatgtactagtgagctgaggcccctgatatggcactgcattcacactgggaagagcagtattttggaaagatgttgggtgtacaggagacagatgactatctggggctatgtttaaagatatttgccgtaccagtgggcctctccttctttctaagagaggcacatgcccagtcactcccactcgagaaggtgaagatggaggctgcaattcagtaagtggtgttgtctggggtggggtgatgcttccacaatcgaatgatttgcttctgagatcagagacctccattgacgtttgcgtgcaattaatctgttctgatgcagtacgcctcatttcccggtgacatccaggaacattcagagtattcaagccagctggaatcataagaaactcggctttatttagaaaatcgattttgggggaagcctccgttttagaaacgtcctctatgtctaaagaggctgagaaacttgaagtgtgagataaactgctctccctacttagactcctggagagagtggaatcaaagctcgattctgttgaggaatgttctatctcagccagacggagccttttctttttgggtggcagtttctctgttggcaattttgacaaggtttcactacgctggggccaactgaacttctctgacttttcttgatcatggcattgagcttccaggtctcgatctggttcttctgtgaccaaaatctctggaacttggatgttgtgctgccggacaagtcttgagggctgtcctaacacatgtcgttcacttggactctttctggagctttcctgaagttctcctctgagagcgtctgatagtgcaagctggtgaggatgagacccgtcccgagaagggtgactttcctcttgggagattcctatcacttttagagacccggacttccccgttctattcagctcctggaaagaaactggggaggctctttcaaaaggctcaggcttgtcaaatgagttgggcctgctcagggagttggtgtgctggatgacagagattccagttccgtgtctctgcagttctatcttgtcctgggctgctgaacttatctgttgttccatgatggtcgacagcttgggatccatggtctgctcagggcccctggcaacaaggtgaatatgggagttttgcaactgtatatttttatgctgctggtcacttcttatggtaacattatgtttaggcaaactgggattacagcccagagcattctgaaactgaaggccttcagaactttttggagatgttccactttcattttgctgaagttcttcatcatccccaacacttttcattttcctcctttttcttatctggggcgtctgttcccagatgccggaggacccagcgactctgtagtgtagaatctgaggctgcagaccgccgggcacagggctgtgctcaggttctctcatggctacctttgtttttggtccatgtaactcagaacagtaaaatttcttatgattttcaaaattttccagtttcctatacctgtttctacaagtttcacactcaaacattgtccctcgcccttgatgagacttctttttttctatatgtgggccttgtgccagtgccttgctcctcactgacatggcttcaccagcagcatggcatccttggtggctctcatccagggactgtccagtaccaagaacatgactttcatttgctgaagagtcttctatggctgcttgtctcacaagtgtacggggatgcccactctggggcacaggagcgttaggtcccgatacaaagacatcatcatagaaagcgccaattttgtcatcaaatgactgacttcctcttagtggatgaggaggaggtattatatttgcaggtactgctgaataacctgtggtcggcatggaattacttcttgtgataggtaaacagtcaagtgaaggtacagacagaagaaacacttgctttgatttttcagtaggggtgaaaggtgacttcggtatatcagagcttgaacttgttctccgtcccactggttttaaatcaaactggaaagaatctttaaatatgtatgatttgggggaatcaatgcttcctcgtcttgacagtgaggttctccgcggcttcacactatccagttgcttgtcatctaccaaagcttcattgtctgagataagcttcgatatccgctcctcaagtgtttttgtggccaaaggtgggcgcatctgacctggtaaaagcaatgccttttcccctgtgggcaaagcagagggtgttgacgtggtgacaagagctgcagagggtccgttactccttccagagtcttgttctgtgctgggtaaccttctggcaaagggagttggtggactcactgtttgatcggcactttcagaacgtgaaaagtaaccagaatccgtacttcctaaacttcgaggactcaggagctttccttgctgctcttgggagtaatcggtagcctgctgcctttgtagctgggcgtgtaccgttcctacgtgagagtcttgctttccttccagtggattcatgtcgcctttctggtgggaattctcattagtctccaacctggagactccaccctgggacatgttggctgaaagtggctgtacgtttgtcacctgaaggtccttctgcttttgtgcactagaaagttcaggcttgggatccatggcctttggactgtcagttcttaagggggacacagtgacatggtggaccacaactttcggtaactctgtcacagcttgtgattctgcagatctgtcctgtagcaaaaagtcacctatcacattttctggactgcttggagtgaagcttgattttagtaaagtttcagcatttgacatcctctttattatgtgcacaggctgcagctccatggcgcccaggtcatgctgtctctcatcagtggcgccttcctcctcgctctccccactgtcttctacgtctgaatgaatactaagtgctttgggggactcgtgggacaagaacaagccaccagcatctggttgcaagacaagacccagtttgatagtatgtgcgtgggatttcttgtgcttatacagattacttttagtcttaaatgaaaatccacaagtcacacagggatagggtcgctctccagtgtgggagcggatatgctttaaaagcacactaggctttgcacatgctctattgcaatactcacaaatatattttccttgtttttttggcttctgatctttcagaagaagattgcacatttgctctacgctttgattaacaacagaggcaacatgagttgaattatagattggcatggggggcgactgtgtagaattagccggacttattgacaaaggtgaagcagaatccatttgctggttttgaggagtaacctgagatctactggaaggtgaagttaggcctacagatgatgtcactgctatattataaacctgttcaagtttggcattctcttgattttgcagatttgtcagtgatcctgtgaaacctgaacaccccggaagctgttgattatgttggttggatttgggaacaaagtgttcatgttgatgatacaaatgagaagctgactgcattgccccttgctcattcttctgagcagcagacatatggactgtgtatgaggtacaagaagactgtgattcagcaaccaattcctgtgaagtctgatttggggcatccattgaactgttttttaatttgggaggggaacgtgcagttttatttggcctcagtttttctgtcttaattgcacaaggtgagcccttttgtgacaaggtgctcagttctggctccattgctttcagtaagacatcgaatgcagtgtttgtataggagggggacgtagtgccacaatgagaagagatgcattcgctattgtcagtcctggttttacttgacaaggaacttgagtcacattgttcatcgaggtcactgaatttggcaggatcagcgccttcggatctccatctacgcagttcagatggttgctgcagaaacaagggcttctttggggagacagattcttcagattttgaggcttcagcaattattccaggtgtttctccattttgtttggtaaactgcttcccattttttacaggaatataattctgtttcttgtgagactccgaagcactatgaagaacggcgaaagatgactcttctgtattttgtttatgttttgcctgaagaggatttctcagtggggattttggtatttttttcaggtgattctcagctacgatctttttgcgtttcacacctttaagggattccgaagttcctttaacaccagcctgtaagatttctttttttgaaacttctgccccattaagttctttttgtgcttcttcaattttgtcaagaccatgcggaagagccaccccgtgcagtccagtgacccttctccacggaacccaggacaacatgctaagcctttcttctgaacaccaagtgctgctctcatgctcttccaaaattcttcaacctcacaaaggataggtcggtgtcaaaacggcacccaccacgtttcctcttagatttctgggatgaatttgtttagttcgaggcatcttctttgactcagggccttctttttcttcttaaaaactgcagataaagcaagccaccaaaaggcagctccataaactcaacatacatcaattaatccatgtgccgaactgcaacacaaaagtctgatccaaagcttcctgggtttaacttttaattttaaaaacaaaaaagcagaaaccaaaagcctcctaggttggaagtgggcgtgagaggaaatgctagagggaggcgcttcattccccgggctgcctgtgcccccctttctggcccctgcccggggctttgatgttatctagtgcaccgcctccatcggtttctaccttgggctctgcgccgccgagaagatagacagatcttccgcacttcacttgcaggttctgagagaggcaagcaggtagtcgcgggaaaggacccacactccttagccccgcagtgagagaggaacatttgcacgggcttcctgttgctacctggactgaaatgaacaatccacccctctagtgatcctggagacttgcaccgtatggtctttcctgctagacgcacagcgggaggcctcctacattagattcattttccctccacccgtagcacaaacttgtaagatggtggtggagtatgtttcctgaggctttgttcgggttttagatctcagtttggaaggtaaatattatttcccttctgagacagtcctgcagcctgtgcctccactttacaccaacagaagcttgtgttcaggccttgccctatgatcgctgagaggcttctgcttgagtagaggacggggtgagcagagtcccatcctgggggtgagttctcagtgggatattgaaggagagaaagttcacgatttggcagtggtggaagtacagcattctagaggagggaaataacttgaaggtgagagcaagtgaactgtgtgtgatggtttttcca

SEQ ID NO: 9711 - RNA, 6229 nt, Homo sapiens
  source 1..6229: mol_type = other RNA
atgcacctgggcaaggattctgatagagaagaattttggctcatctctgaaaaaacattttcacatagaaattccttctctgggtttggcaaagcattctgatgacctttttgtaatgttggcacagaattttgttcttcactgattggcactacactatgattagtctggcaaattggctgattgggcagatcttgggtcactagtatttgtggcagggatgtgagtgtagcaaaacagtaagcaggaacactactctgcaggcgtatgggcagcatgaatgatgatggcaccttctgcacctgacttccaaggggcctgagctctggtggtagcagaggatgcgaattagacatgctgtcaattaatttggttggtaatgttgctgatgtcacacaatgatctgttccaactggatctgaaataacttgatttggcaaagaatgcacaggattagaagagcaagatgggcctgaagtgaaaacctgacaatgcaattggtatttgggagcaaagcaatcctcacttttagaagacccagataaaacagaatttttatctggcttgctaccctgcgtagacacttgcagagatagctgtgtgctctggtggctaggcggtgcatggatttgatttaacaaattgatatcacagagctgttgaacaggaaaaacgttggtagagctggagtttgatgtttctgcctgcagatccttaacctgagtctgagagtgcaaagtatttgcagaaaactcagctaaagatgtactagtgagctgaggcccctgatatggcactgcattcacactgggaagagcagtattttggaaagatgttgggtgtacaggagacagatgactatctggggctatgtttaaagatatttgccgtaccagtgggcctctccttctttctaagagaggcacatgcccagtcactcccactcgagaaggtgaagatggaggctgcaattcagtaagtggtgttgtctggggtggggtgatgcttccacaatcgaatgatttgcttctgagatcagagacctccattgacgtttgcgtgcaattaatctgttctgatgcagtacgcctcatttcccggtgacatccaggaacattcagagtattcaagccagctggaatcataagaaactcggctttatttagaaaatcgattttgggggaagcctccgttttagaaacgtcctctatgtctaaagaggctgagaaacttgaagtgtgagataaactgctctccctacttagactcctggagagagtggaatcaaagctcgattctgttgaggaatgttctatctcagccagacggagccttttctttttgggtggcagtttctctgttggcaattttgacaaggtttcactacgctggggccaactgaacttctctgacttttcttgatcatggcattgagcttccaggtctcgatctggttcttctgtgaccaaaatctctggaacttggatgttgtgctgccggacaagtcttgagggctgtcctaacacatgtcgttcacttggactctttctggagctttcctgaagttctcctctgagagcgtctgatagtgcaagctggtgaggatgagacccgtcccgagaagggtgactttcctcttgggagattcctatcacttttagagacccggacttccccgttctattcagctcctggaaagaaactggggaggctctttcaaaaggctcaggcttgtcaaatgagttgggcctgctcagggagttggtgtgctggatgacagagattccagttccgtgtctctgcagttctatcttgtcctgggctgctgaacttatctgttgttccatgatggtcgacagcttgggatccatggtctgctcagggcccctggcaacaaggtgaatatgggagttttgcaactgtatatttttatgctgctggtcacttcttatggtaacattatgtttaggcaaactgggattacagcccagagcattctgaaactgaaggccttcagaactttttggagatgttccactttcattttgctgaagttcttcatcatccccaacacttttcattttcctcctttttcttatctggggcgtctgttcccagatgccggaggacccagcgactctgtagtgtagaatctgaggctgcagaccgccgggcacagggctgtgctcaggttctctcatggctacctttgtttttggtccatgtaactcagaacagtaaaatttcttatgattttcaaaattttccagtttcctatacctgtttctacaagtttcacactcaaacattgtccctcgcccttgatgagacttctttttttctatatgtgggccttgtgccagtgccttgctcctcactgacatggcttcaccagcagcatggcatccttggtggctctcatccagggactgtccagtaccaagaacatgactttcatttgctgaagagtcttctatggctgcttgtctcacaagtgtacggggatgcccactctggggcacaggagcgttaggtcccgatacaaagacatcatcatagaaagcgccaattttgtcatcaaatgactgacttcctcttagtggatgaggaggaggtattatatttgcaggtactgctgaataacctgtggtcggcatggaattacttcttgtgataggtaaacagtcaagtgaaggtacagacagaagaaacacttgctttgatttttcagtaggggtgaaaggtgacttcggtatatcagagcttgaacttgttctccgtcccactggttttaaatcaaactggaaagaatctttaaatatgtatgatttgggggaatcaatgcttcctcgtcttgacagtgaggttctccgcggcttcacactatccagttgcttgtcatctaccaaagcttcattgtctgagataagcttcgatatccgctcctcaagtgtttttgtggccaaaggtgggcgcatctgacctggtaaaagcaatgccttttcccctgtgggcaaagcagagggtgttgacgtggtgacaagagctgcagagggtccgttactccttccagagtcttgttctgtgctgggtaaccttctggcaaagggagttggtggactcactgtttgatcggcactttcagaacgtgaaaagtaaccagaatccgtacttcctaaacttcgaggactcaggagctttccttgctgctcttgggagtaatcggtagcctgctgcctttgtagctgggcgtgtaccgttcctacgtgagagtcttgctttccttccagtggattcatgtcgcctttctggtgggaattctcattagtctccaacctggagactccaccctgggacatgttggctgaaagtggctgtacgtttgtcacctgaaggtccttctgcttttgtgcactagaaagttcaggcttgggatccatggcctttggactgtcagttcttaagggggacacagtgacatggtggaccacaactttcggtaactctgtcacagcttgtgattctgcagatctgtcctgtagcaaaaagtcacctatcacattttctggactgcttggagtgaagcttgattttagtaaagtttcagcatttgacatcctctttattatgtgcacaggctgcagctccatggcgcccaggtcatgctgtctctcatcagtggcgccttcctcctcgctctccccactgtcttctacgtctgaatgaatactaagtgctttgggggactcgtgggacaagaacaagccaccagcatctggttgcaagacaagacccagtttgatagtatgtgcgtgggatttcttgtgcttatacagattacttttagtcttaaatgaaaatccacaagtcacacagggatagggtcgctctccagtgtgggagcggatatgctttaaaagcacactaggctttgcacatgctctattgcaatactcacaaatatattttccttgtttttttggcttctgatctttcagaagaagattgcacatttgctctacgctttgattaacaacagaggcaacatgagttgaattatagattggcatggggggcgactgtgtagaattagccggacttattgacaaaggtgaagcagaatccatttgctggttttgaggagtaacctgagatctactggaaggtgaagttaggcctacagatgatgtcactgctatattataaacctgttcaagtttggcattctcttgattttgcagatttgtcagtgatcctgtgaaacctgaacaccccggaagctgttgattatgttggttggatttgggaacaaagtgttcatgttgatgatacaaatgagaagctgactgcattgccccttgctcattcttctgagcagcagacatatggactgtgtatgaggtacaagaagactgtgattcagcaaccaattcctgtgaagtctgatttggggcatccattgaactgttttttaatttgggaggggaacgtgcagttttatttggcctcagtttttctgtcttaattgcacaaggtgagcccttttgtgacaaggtgctcagttctggctccattgctttcagtaagacatcgaatgcagtgtttgtataggagggggacgtagtgccacaatgagaagagatgcattcgctattgtcagtcctggttttacttgacaaggaacttgagtcacattgttcatcgaggtcactgaatttggcaggatcagcgccttcggatctccatctacgcagttcagatggttgctgcagaaacaagggcttctttggggagacagattcttcagattttgaggcttcagcaattattccaggtgtttctccattttgtttggtaaactgcttcccattttttacaggaatataattctgtttcttgtgagactccgaagcactatgaagaacggcgaaagatgactcttctgtattttgtttatgttttgcctgaagaggatttctcagtggggattttggtatttttttcaggtgattctcagctacgatctttttgcgtttcacacctttaagggattccgaagttcctttaacaccagcctgtaagatttctttttttgaaacttctgccccattaagttctttttgtgcttcttcaattttgtcaagaccatgcggaagagccaccccgtgcagtccagtgacccttctccacggaacccaggacaacatgctaagcctttcttctgaacaccaagtgctgctctcatgctcttccaaaattcttcaacctcacaaaggataggtcggtgtcaaaacggcacccaccacgtttcctcttagatttctgggatgaatttgtttagttcgaggcatcttctttgactcagggccttctttttcttcttaaaaactgcagataaagcaagccaccaaaaggcagctccataaactcaacatacatcaattaatccatgtgccgaactgcaacacaaaagtctgatccaaagcttcctgggtttaacttttaattttaaaaacaaaaaagcagaaaccaaaagcctcctaggttggaagtgggcgtgagaggaaatgctagagggaggcgcttcattccccgggctgcctgtgcccccctttctggcccctgcccggggctttgatgttatctagtgcaccgcctccatcggtttctaccttgggctctgcgccgccgagaagatagacagatcttccgcacttcacttgcaggttctgagagaggcaagcaggtagtcgcgggaaaggacccacactccttagccccgcagtgagagaggaacatttgcacgggcttcctgttgctacctggactgaaatgaacaatccacccctctagtgatcctggagacttgcaccgtatggtctttcctgctagacgcacagcgggaggcctcctacattagattcattttccctccacccgtagcacaaacttgtaagatggtggtggagtatgtttcctgaggctttgttcgggttttagatctcagtttggaaggtaaatattatttcccttctgagacagtcctgcagcctgtgcctccactttacaccaacagaagcttgtgttcaggccttgccctctggaagattacaaattaatggagacaggataaacacatggaaaaataccagcttctgactctgtaagtatgttgccaacataagaagctttctccagatgcctgttcatgggatcaaattttgcagat

SEQ ID NO: 9712 - RNA, 6402 nt, Homo sapiens
  source 1..6402: mol_type = other RNA
atgcacctgggcaaggattctgatagagaagaattttggctcatctctgaaaaaacattttcacatagaaattccttctctgggtttggcaaagcattctgatgacctttttgtaatgttggcacagaattttgttcttcactgattggcactacactatgattagtctggcaaattggctgattgggcagatcttgggtcactagtatttgtggcagggatgtgagtgtagcaaaacagtaagcaggaacactactctgcaggcgtatgggcagcatgaatgatgatggcaccttctgcacctgacttccaaggggcctgagctctggtggtagcagaggatgcgaattagacatgctgtcaattaatttggttggtaatgttgctgatgtcacacaatgatctgttccaactggatctgaaataacttgatttggcaaagaatgcacaggattagaagagcaagatgggcctgaagtgaaaacctgacaatgcaattggtatttgggagcaaagcaatcctcacttttagaagacccagataaaacagaatttttatctggcttgctaccctgcgtagacacttgcagagatagctgtgtgctctggtggctaggcggtgcatggatttgatttaacaaattgatatcacagagctgttgaacaggaaaaacgttggtagagctggagtttgatgtttctgcctgcagatccttaacctgagtctgagagtgcaaagtatttgcagaaaactcagctaaagatgtactagtgagctgaggcccctgatatggcactgcattcacactgggaagagcagtattttggaaagatgttgggtgtacaggagacagatgactatctggggctatgtttaaagatatttgccgtaccagtgggcctctccttctttctaagagaggcacatgcccagtcactcccactcgagaaggtgaagatggaggctgcaattcagtaagtggtgttgtctggggtggggtgatgcttccacaatcgaatgatttgcttctgagatcagagacctccattgacgtttgcgtgcaattaatctgttctgatgcagtacgcctcatttcccggtgacatccaggaacattcagagtattcaagccagctggaatcataagaaactcggctttatttagaaaatcgattttgggggaagcctccgttttagaaacgtcctctatgtctaaagaggctgagaaacttgaagtgtgagataaactgctctccctacttagactcctggagagagtggaatcaaagctcgattctgttgaggaatgttctatctcagccagacggagccttttctttttgggtggcagtttctctgttggcaattttgacaaggtttcactacgctggggccaactgaacttctctgacttttcttgatcatggcattgagcttccaggtctcgatctggttcttctgtgaccaaaatctctggaacttggatgttgtgctgccggacaagtcttgagggctgtcctaacacatgtcgttcacttggactctttctggagctttcctgaagttctcctctgagagcgtctgatagtgcaagctggtgaggatgagacccgtcccgagaagggtgactttcctcttgggagattcctatcacttttagagacccggacttccccgttctattcagctcctggaaagaaactggggaggctctttcaaaaggctcaggcttgtcaaatgagttgggcctgctcagggagttggtgtgctggatgacagagattccagttccgtgtctctgcagttctatcttgtcctgggctgctgaacttatctgttgttccatgatggtcgacagcttgggatccatggtctgctcagggcccctggcaacaaggtgaatatgggagttttgcaactgtatatttttatgctgctggtcacttcttatggtaacattatgtttaggcaaactgggattacagcccagagcattctgaaactgaaggccttcagaactttttggagatgttccactttcattttgctgaagttcttcatcatccccaacacttttcattttcctcctttttcttatctggggcgtctgttcccagatgccggaggacccagcgactctgtagtgtagaatctgaggctgcagaccgccgggcacagggctgtgctcaggttctctcatggctacctttgtttttggtccatgtaactcagaacagtaaaatttcttatgattttcaaaattttccagtttcctatacctgtttctacaagtttcacactcaaacattgtccctcgcccttgatgagacttctttttttctatatgtgggccttgtgccagtgccttgctcctcactgacatggcttcaccagcagcatggcatccttggtggctctcatccagggactgtccagtaccaagaacatgactttcatttgctgaagagtcttctatggctgcttgtctcacaagtgtacggggatgcccactctggggcacaggagcgttaggtcccgatacaaagacatcatcatagaaagcgccaattttgtcatcaaatgactgacttcctcttagtggatgaggaggaggtattatatttgcaggtactgctgaataacctgtggtcggcatggaattacttcttgtgataggtaaacagtcaagtgaaggtacagacagaagaaacacttgctttgatttttcagtaggggtgaaaggtgacttcggtatatcagagcttgaacttgttctccgtcccactggttttaaatcaaactggaaagaatctttaaatatgtatgatttgggggaatcaatgcttcctcgtcttgacagtgaggttctccgcggcttcacactatccagttgcttgtcatctaccaaagcttcattgtctgagataagcttcgatatccgctcctcaagtgtttttgtggccaaaggtgggcgcatctgacctggtaaaagcaatgccttttcccctgtgggcaaagcagagggtgttgacgtggtgacaagagctgcagagggtccgttactccttccagagtcttgttctgtgctgggtaaccttctggcaaagggagttggtggactcactgtttgatcggcactttcagaacgtgaaaagtaaccagaatccgtacttcctaaacttcgaggactcaggagctttccttgctgctcttgggagtaatcggtagcctgctgcctttgtagctgggcgtgtaccgttcctacgtgagagtcttgctttccttccagtggattcatgtcgcctttctggtgggaattctcattagtctccaacctggagactccaccctgggacatgttggctgaaagtggctgtacgtttgtcacctgaaggtccttctgcttttgtgcactagaaagttcaggcttgggatccatggcctttggactgtcagttcttaagggggacacagtgacatggtggaccacaactttcggtaactctgtcacagcttgtgattctgcagatctgtcctgtagcaaaaagtcacctatcacattttctggactgcttggagtgaagcttgattttagtaaagtttcagcatttgacatcctctttattatgtgcacaggctgcagctccatggcgcccaggtcatgctgtctctcatcagtggcgccttcctcctcgctctccccactgtcttctacgtctgaatgaatactaagtgctttgggggactcgtgggacaagaacaagccaccagcatctggttgcaagacaagacccagtttgatagtatgtgcgtgggatttcttgtgcttatacagattacttttagtcttaaatgaaaatccacaagtcacacagggatagggtcgctctccagtgtgggagcggatatgctttaaaagcacactaggctttgcacatgctctattgcaatactcacaaatatattttccttgtttttttggcttctgatctttcagaagaagattgcacatttgctctacgctttgattaacaacagaggcaacatgagttgaattatagattggcatggggggcgactgtgtagaattagccggacttattgacaaaggtgaagcagaatccatttgctggttttgaggagtaacctgagatctactggaaggtgaagttaggcctacagatgatgtcactgctatattataaacctgttcaagtttggcattctcttgattttgcagatttgtcagtgatcctgtgaaacctgaacaccccggaagctgttgattatgttggttggatttgggaacaaagtgttcatgttgatgatacaaatgagaagctgactgcattgccccttgctcattcttctgagcagcagacatatggactgtgtatgaggtacaagaagactgtgattcagcaaccaattcctgtgaagtctgatttggggcatccattgaactgttttttaatttgggaggggaacgtgcagttttatttggcctcagtttttctgtcttaattgcacaaggtgagcccttttgtgacaaggtgctcagttctggctccattgctttcagtaagacatcgaatgcagtgtttgtataggagggggacgtagtgccacaatgagaagagatgcattcgctattgtcagtcctggttttacttgacaaggaacttgagtcacattgttcatcgaggtcactgaatttggcaggatcagcgccttcggatctccatctacgcagttcagatggttgctgcagaaacaagggcttctttggggagacagattcttcagattttgaggcttcagcaattattccaggtgtttctccattttgtttggtaaactgcttcccattttttacaggaatataattctgtttcttgtgagactccgaagcactatgaagaacggcgaaagatgactcttctgtattttgtttatgttttgcctgaagaggatttctcagtggggattttggtatttttttcaggtgattctcagctacgatctttttgcgtttcacacctttaagggattccgaagttcctttaacaccagcctgtaagatttctttttttgaaacttctgccccattaagttctttttgtgcttcttcaattttgtcaagaccatgcggaagagccaccccgtgcagtccagtgacccttctccacggaacccaggacaacatgctaagcctttcttctgaacaccaagtgctgctctcatgctcttccaaaattcttcaacctcacaaaggataggtcggtgtcaaaacggcacccaccacgtttcctcttagatttctgggatgaatttgtttagttcgaggcatcttctttgactcagggccttctttttcttcttaaaaactgcagataaagcaagccaccaaaaggcagctccataaactcaacatacatcaattaatccatgtgccgaactgcaacacaaaagtctgatccaaagcttcctgggtttaacttttaattttaaaaacaaaaaagcagaaaccaaaagcctcctaggttggaagtgggcgtgagaggaaatgctagagggaggcgcttcattccccgggctgcctgtgcccccctttctggcccctgcccggggctttgatgttatctagtgcaccgcctccatcggtttctaccttgggctctgcgccgccgagaagatagacagatcttccgcacttcacttgcaggttctgagagaggcaagcaggtagtcgcgggaaaggacccacactccttagccccgcagtgagagaggaacatttgcacgggcttcctgttgctacctggactgaaatgaacaatccacccctctagtgatcctggagacttgcaccgtatggtctttcctgctagacgcacagcgggaggcctcctacattagattcattttccctccacccgtagcacaaacttgtaagatggtggtggagtatgtttcctgaggctttgttcgggttttagatctcagtttggaaggtaaatattatttcccttctgagacagtcctgcagcctgtgcctccactttacaccaacagaagcttgtgttcaggccttgccctctggaagattacaaattaatggagacaggataaacacatggaaaaatacctagagggaaaaaaagatataagaggcttataaacagagccaattaaagttatacagttatttacatgatcgctgagaggcttctgcttgagtagaggacggggtgagcagagtcccatcctgggggtgagttctcagtgggatattgaaggagagaaagttcacgatttggcagtggtggaagtacagcattctagaggagggaaataacttgaaggtgagagcaagtgaactgtgtgtgatggtttttcca

SEQ ID NO: 9713 - RNA, 6403 nt, Homo sapiens
  source 1..6403: mol_type = other RNA
atgcacctgggcaaggattctgatagagaagaattttggctcatctctgaaaaaacattttcacatagaaattccttctctgggtttggcaaagcattctgatgacctttttgtaatgttggcacagaattttgttcttcactgattggcactacactatgattagtctggcaaattggctgattgggcagatcttgggtcactagtatttgtggcagggatgtgagtgtagcaaaacagtaagcaggaacactactctgcaggcgtatgggcagcatgaatgatgatggcaccttctgcacctgacttccaaggggcctgagctctggtggtagcagaggatgcgaattagacatgctgtcaattaatttggttggtaatgttgctgatgtcacacaatgatctgttccaactggatctgaaataacttgatttggcaaagaatgcacaggattagaagagcaagatgggcctgaagtgaaaacctgacaatgcaattggtatttgggagcaaagcaatcctcacttttagaagacccagataaaacagaatttttatctggcttgctaccctgcgtagacacttgcagagatagctgtgtgctctggtggctaggcggtgcatggatttgatttaacaaattgatatcacagagctgttgaacaggaaaaacgttggtagagctggagtttgatgtttctgcctgcagatccttaacctgagtctgagagtgcaaagtatttgcagaaaactcagctaaagatgtactagtgagctgaggcccctgatatggcactgcattcacactgggaagagcagtattttggaaagatgttgggtgtacaggagacagatgactatctggggctatgtttaaagatatttgccgtaccagtgggcctctccttctttctaagagaggcacatgcccagtcactcccactcgagaaggtgaagatggaggctgcaattcagtaagtggtgttgtctggggtggggtgatgcttccacaatcgaatgatttgcttctgagatcagagacctccattgacgtttgcgtgcaattaatctgttctgatgcagtacgcctcatttcccggtgacatccaggaacattcagagtattcaagccagctggaatcataagaaactcggctttatttagaaaatcgattttgggggaagcctccgttttagaaacgtcctctatgtctaaagaggctgagaaacttgaagtgtgagataaactgctctccctacttagactcctggagagagtggaatcaaagctcgattctgttgaggaatgttctatctcagccagacggagccttttctttttgggtggcagtttctctgttggcaattttgacaaggtttcactacgctggggccaactgaacttctctgacttttcttgatcatggcattgagcttccaggtctcgatctggttcttctgtgaccaaaatctctggaacttggatgttgtgctgccggacaagtcttgagggctgtcctaacacatgtcgttcacttggactctttctggagctttcctgaagttctcctctgagagcgtctgatagtgcaagctggtgaggatgagacccgtcccgagaagggtgactttcctcttgggagattcctatcacttttagagacccggacttccccgttctattcagctcctggaaagaaactggggaggctctttcaaaaggctcaggcttgtcaaatgagttgggcctgctcagggagttggtgtgctggatgacagagattccagttccgtgtctctgcagttctatcttgtcctgggctgctgaacttatctgttgttccatgatggtcgacagcttgggatccatggtctgctcagggcccctggcaacaaggtgaatatgggagttttgcaactgtatatttttatgctgctggtcacttcttatggtaacattatgtttaggcaaactgggattacagcccagagcattctgaaactgaaggccttcagaactttttggagatgttccactttcattttgctgaagttcttcatcatccccaacacttttcattttcctcctttttcttatctggggcgtctgttcccagatgccggaggacccagcgactctgtagtgtagaatctgaggctgcagaccgccgggcacagggctgtgctcaggttctctcatggctacctttgtttttggtccatgtaactcagaacagtaaaatttcttatgattttcaaaattttccagtttcctatacctgtttctacaagtttcacactcaaacattgtccctcgcccttgatgagacttctttttttctatatgtgggccttgtgccagtgccttgctcctcactgacatggcttcaccagcagcatggcatccttggtggctctcatccagggactgtccagtaccaagaacatgactttcatttgctgaagagtcttctatggctgcttgtctcacaagtgtacggggatgcccactctggggcacaggagcgttaggtcccgatacaaagacatcatcatagaaagcgccaattttgtcatcaaatgactgacttcctcttagtggatgaggaggaggtattatatttgcaggtactgctgaataacctgtggtcggcatggaattacttcttgtgataggtaaacagtcaagtgaaggtacagacagaagaaacacttgctttgatttttcagtaggggtgaaaggtgacttcggtatatcagagcttgaacttgttctccgtcccactggttttaaatcaaactggaaagaatctttaaatatgtatgatttgggggaatcaatgcttcctcgtcttgacagtgaggttctccgcggcttcacactatccagttgcttgtcatctaccaaagcttcattgtctgagataagcttcgatatccgctcctcaagtgtttttgtggccaaaggtgggcgcatctgacctggtaaaagcaatgccttttcccctgtgggcaaagcagagggtgttgacgtggtgacaagagctgcagagggtccgttactccttccagagtcttgttctgtgctgggtaaccttctggcaaagggagttggtggactcactgtttgatcggcactttcagaacgtgaaaagtaaccagaatccgtacttcctaaacttcgaggactcaggagctttccttgctgctcttgggagtaatcggtagcctgctgcctttgtagctgggcgtgtaccgttcctacgtgagagtcttgctttccttccagtggattcatgtcgcctttctggtgggaattctcattagtctccaacctggagactccaccctgggacatgttggctgaaagtggctgtacgtttgtcacctgaaggtccttctgcttttgtgcactagaaagttcaggcttgggatccatggcctttggactgtcagttcttaagggggacacagtgacatggtggaccacaactttcggtaactctgtcacagcttgtgattctgcagatctgtcctgtagcaaaaagtcacctatcacattttctggactgcttggagtgaagcttgattttagtaaagtttcagcatttgacatcctctttattatgtgcacaggctgcagctccatggcgcccaggtcatgctgtctctcatcagtggcgccttcctcctcgctctccccactgtcttctacgtctgaatgaatactaagtgctttgggggactcgtgggacaagaacaagccaccagcatctggttgcaagacaagacccagtttgatagtatgtgcgtgggatttcttgtgcttatacagattacttttagtcttaaatgaaaatccacaagtcacacagggatagggtcgctctccagtgtgggagcggatatgctttaaaagcacactaggctttgcacatgctctattgcaatactcacaaatatattttccttgtttttttggcttctgatctttcagaagaagattgcacatttgctctacgctttgattaacaacagaggcaacatgagttgaattatagattggcatggggggcgactgtgtagaattagccggacttattgacaaaggtgaagcagaatccatttgctggttttgaggagtaacctgagatctactggaaggtgaagttaggcctacagatgatgtcactgctatattataaacctgttcaagtttggcattctcttgattttgcagatttgtcagtgatcctgtgaaacctgaacaccccggaagctgttgattatgttggttggatttgggaacaaagtgttcatgttgatgatacaaatgagaagctgactgcattgccccttgctcattcttctgagcagcagacatatggactgtgtatgaggtacaagaagactgtgattcagcaaccaattcctgtgaagtctgatttggggcatccattgaactgttttttaatttgggaggggaacgtgcagttttatttggcctcagtttttctgtcttaattgcacaaggtgagcccttttgtgacaaggtgctcagttctggctccattgctttcagtaagacatcgaatgcagtgtttgtataggagggggacgtagtgccacaatgagaagagatgcattcgctattgtcagtcctggttttacttgacaaggaacttgagtcacattgttcatcgaggtcactgaatttggcaggatcagcgccttcggatctccatctacgcagttcagatggttgctgcagaaacaagggcttctttggggagacagattcttcagattttgaggcttcagcaattattccaggtgtttctccattttgtttggtaaactgcttcccattttttacaggaatataattctgtttcttgtgagactccgaagcactatgaagaacggcgaaagatgactcttctgtattttgtttatgttttgcctgaagaggatttctcagtggggattttggtatttttttcaggtgattctcagctacgatctttttgcgtttcacacctttaagggattccgaagttcctttaacaccagcctgtaagatttctttttttgaaacttctgccccattaagttctttttgtgcttcttcaattttgtcaagaccatgcggaagagccaccccgtgcagtccagtgacccttctccacggaacccaggacaacatgctaagcctttcttctgaacaccaagtgctgctctcatgctcttccaaaattcttcaacctcacaaaggataggtcggtgtcaaaacggcacccaccacgtttcctcttagatttctgggatgaatttgtttagttcgaggcatcttctttgactcagggccttctttttcttcttaaaaactgcagataaagcaagccaccaaaaggcagctccataaactcaacatacatcaattaatccatgtgccgaactgcaacacaaaagtctgatccaaagcttcctgggtttaacttttaattttaaaaacaaaaaagcagaaaccaaaagcctcctaggttggaagtgggcgtgagaggaaatgctagagggaggcgcttcattccccgggctgcctgtgcccccctttctggcccctgcccggggctttgatgttatctagtgcaccgcctccatcggtttctaccttgggctctgcgccgccgagaagatagacagatcttccgcacttcacttgcaggttctgagagaggcaagcaggtagtcgcgggaaaggacccacactccttagccccgcagtgagagaggaacatttgcacgggcttcctgttgctacctggactgaaatgaacaatccacccctctagtgatcctggagacttgcaccgtatggtctttcctgctagacgcacagcgggaggcctcctacattagattcattttccctccacccgtagcacaaacttgtaagatggtggtggagtatgtttcctgaggctttgttcgggttttagatctcagtttggaaggtaaatattatttcccttctgagacagtcctgcagcctgtgcctccactttacaccaacagaagcttgtgttcaggccttgccctctggaagattacaaattaatggagacaggataaacacatggaaaaatacctagagggaaaaaaagatataagaggcttataaacagagccaattaaagttatacagttatttacatgatcgctgagaggcttctgcttgagtagaggacggggtgagcagagtcccatcctgggggtgagttctcagtgggatattgaaggagagaaagttcacgatttggcagtggtggaagtacagcattctagaggagggaaataacttgaaggtgagagcaagtgaactgtgtgtgatggtttttccac

SEQ ID NO: 9714 - RNA, 6405 nt, Homo sapiens
  source 1..6405: mol_type = other RNA
atgcacctgggcaaggattctgatagagaagaattttggctcatctctgaaaaaacattttcacatagaaattccttctctgggtttggcaaagcattctgatgacctttttgtaatgttggcacagaattttgttcttcactgattggcactacactatgattagtctggcaaattggctgattgggcagatcttgggtcactagtatttgtggcagggatgtgagtgtagcaaaacagtaagcaggaacactactctgcaggcgtatgggcagcatgaatgatgatggcaccttctgcacctgacttccaaggggcctgagctctggtggtagcagaggatgcgaattagacatgctgtcaattaatttggttggtaatgttgctgatgtcacacaatgatctgttccaactggatctgaaataacttgatttggcaaagaatgcacaggattagaagagcaagatgggcctgaagtgaaaacctgacaatgcaattggtatttgggagcaaagcaatcctcacttttagaagacccagataaaacagaatttttatctggcttgctaccctgcgtagacacttgcagagatagctgtgtgctctggtggctaggcggtgcatggatttgatttaacaaattgatatcacagagctgttgaacaggaaaaacgttggtagagctggagtttgatgtttctgcctgcagatccttaacctgagtctgagagtgcaaagtatttgcagaaaactcagctaaagatgtactagtgagctgaggcccctgatatggcactgcattcacactgggaagagcagtattttggaaagatgttgggtgtacaggagacagatgactatctggggctatgtttaaagatatttgccgtaccagtgggcctctccttctttctaagagaggcacatgcccagtcactcccactcgagaaggtgaagatggaggctgcaattcagtaagtggtgttgtctggggtggggtgatgcttccacaatcgaatgatttgcttctgagatcagagacctccattgacgtttgcgtgcaattaatctgttctgatgcagtacgcctcatttcccggtgacatccaggaacattcagagtattcaagccagctggaatcataagaaactcggctttatttagaaaatcgattttgggggaagcctccgttttagaaacgtcctctatgtctaaagaggctgagaaacttgaagtgtgagataaactgctctccctacttagactcctggagagagtggaatcaaagctcgattctgttgaggaatgttctatctcagccagacggagccttttctttttgggtggcagtttctctgttggcaattttgacaaggtttcactacgctggggccaactgaacttctctgacttttcttgatcatggcattgagcttccaggtctcgatctggttcttctgtgaccaaaatctctggaacttggatgttgtgctgccggacaagtcttgagggctgtcctaacacatgtcgttcacttggactctttctggagctttcctgaagttctcctctgagagcgtctgatagtgcaagctggtgaggatgagacccgtcccgagaagggtgactttcctcttgggagattcctatcacttttagagacccggacttccccgttctattcagctcctggaaagaaactggggaggctctttcaaaaggctcaggcttgtcaaatgagttgggcctgctcagggagttggtgtgctggatgacagagattccagttccgtgtctctgcagttctatcttgtcctgggctgctgaacttatctgttgttccatgatggtcgacagcttgggatccatggtctgctcagggcccctggcaacaaggtgaatatgggagttttgcaactgtatatttttatgctgctggtcacttcttatggtaacattatgtttaggcaaactgggattacagcccagagcattctgaaactgaaggccttcagaactttttggagatgttccactttcattttgctgaagttcttcatcatccccaacacttttcattttcctcctttttcttatctggggcgtctgttcccagatgccggaggacccagcgactctgtagtgtagaatctgaggctgcagaccgccgggcacagggctgtgctcaggttctctcatggctacctttgtttttggtccatgtaactcagaacagtaaaatttcttatgattttcaaaattttccagtttcctatacctgtttctacaagtttcacactcaaacattgtccctcgcccttgatgagacttctttttttctatatgtgggccttgtgccagtgccttgctcctcactgacatggcttcaccagcagcatggcatccttggtggctctcatccagggactgtccagtaccaagaacatgactttcatttgctgaagagtcttctatggctgcttgtctcacaagtgtacggggatgcccactctggggcacaggagcgttaggtcccgatacaaagacatcatcatagaaagcgccaattttgtcatcaaatgactgacttcctcttagtggatgaggaggaggtattatatttgcaggtactgctgaataacctgtggtcggcatggaattacttcttgtgataggtaaacagtcaagtgaaggtacagacagaagaaacacttgctttgatttttcagtaggggtgaaaggtgacttcggtatatcagagcttgaacttgttctccgtcccactggttttaaatcaaactggaaagaatctttaaatatgtatgatttgggggaatcaatgcttcctcgtcttgacagtgaggttctccgcggcttcacactatccagttgcttgtcatctaccaaagcttcattgtctgagataagcttcgatatccgctcctcaagtgtttttgtggccaaaggtgggcgcatctgacctggtaaaagcaatgccttttcccctgtgggcaaagcagagggtgttgacgtggtgacaagagctgcagagggtccgttactccttccagagtcttgttctgtgctgggtaaccttctggcaaagggagttggtggactcactgtttgatcggcactttcagaacgtgaaaagtaaccagaatccgtacttcctaaacttcgaggactcaggagctttccttgctgctcttgggagtaatcggtagcctgctgcctttgtagctgggcgtgtaccgttcctacgtgagagtcttgctttccttccagtggattcatgtcgcctttctggtgggaattctcattagtctccaacctggagactccaccctgggacatgttggctgaaagtggctgtacgtttgtcacctgaaggtccttctgcttttgtgcactagaaagttcaggcttgggatccatggcctttggactgtcagttcttaagggggacacagtgacatggtggaccacaactttcggtaactctgtcacagcttgtgattctgcagatctgtcctgtagcaaaaagtcacctatcacattttctggactgcttggagtgaagcttgattttagtaaagtttcagcatttgacatcctctttattatgtgcacaggctgcagctccatggcgcccaggtcatgctgtctctcatcagtggcgccttcctcctcgctctccccactgtcttctacgtctgaatgaatactaagtgctttgggggactcgtgggacaagaacaagccaccagcatctggttgcaagacaagacccagtttgatagtatgtgcgtgggatttcttgtgcttatacagattacttttagtcttaaatgaaaatccacaagtcacacagggatagggtcgctctccagtgtgggagcggatatgctttaaaagcacactaggctttgcacatgctctattgcaatactcacaaatatattttccttgtttttttggcttctgatctttcagaagaagattgcacatttgctctacgctttgattaacaacagaggcaacatgagttgaattatagattggcatggggggcgactgtgtagaattagccggacttattgacaaaggtgaagcagaatccatttgctggttttgaggagtaacctgagatctactggaaggtgaagttaggcctacagatgatgtcactgctatattataaacctgttcaagtttggcattctcttgattttgcagatttgtcagtgatcctgtgaaacctgaacaccccggaagctgttgattatgttggttggatttgggaacaaagtgttcatgttgatgatacaaatgagaagctgactgcattgccccttgctcattcttctgagcagcagacatatggactgtgtatgaggtacaagaagactgtgattcagcaaccaattcctgtgaagtctgatttggggcatccattgaactgttttttaatttgggaggggaacgtgcagttttatttggcctcagtttttctgtcttaattgcacaaggtgagcccttttgtgacaaggtgctcagttctggctccattgctttcagtaagacatcgaatgcagtgtttgtataggagggggacgtagtgccacaatgagaagagatgcattcgctattgtcagtcctggttttacttgacaaggaacttgagtcacattgttcatcgaggtcactgaatttggcaggatcagcgccttcggatctccatctacgcagttcagatggttgctgcagaaacaagggcttctttggggagacagattcttcagattttgaggcttcagcaattattccaggtgtttctccattttgtttggtaaactgcttcccattttttacaggaatataattctgtttcttgtgagactccgaagcactatgaagaacggcgaaagatgactcttctgtattttgtttatgttttgcctgaagaggatttctcagtggggattttggtatttttttcaggtgattctcagctacgatctttttgcgtttcacacctttaagggattccgaagttcctttaacaccagcctgtaagatttctttttttgaaacttctgccccattaagttctttttgtgcttcttcaattttgtcaagaccatgcggaagagccaccccgtgcagtccagtgacccttctccacggaacccaggacaacatgctaagcctttcttctgaacaccaagtgctgctctcatgctcttccaaaattcttcaacctcacaaaggataggtcggtgtcaaaacggcacccaccacgtttcctcttagatttctgggatgaatttgtttagttcgaggcatcttctttgactcagggccttctttttcttcttaaaaactgcagataaagcaagccaccaaaaggcagctccataaactcaacatacatcaattaatccatgtgccgaactgcaacacaaaagtctgatccaaagcttcctgggtttaacttttaattttaaaaacaaaaaagcagaaaccaaaagcctcctaggttggaagtgggcgtgagaggaaatgctagagggaggcgcttcattccccgggctgcctgtgcccccctttctggcccctgcccggggctttgatgttatctagtgcaccgcctccatcggtttctaccttgggctctgcgccgccgagaagatagacagatcttccgcacttcacttgcaggttctgagagaggcaagcaggtagtcgcgggaaaggacccacactccttagccccgcagtgagagaggaacatttgcacgggcttcctgttgctacctggactgaaatgaacaatccacccctctagtgatcctggagacttgcaccgtatggtctttcctgctagacgcacagcgggaggcctcctacattagattcattttccctccacccgtagcacaaacttgtaagatggtggtggagtatgtttcctgaggctttgttcgggttttagatctcagtttggaaggtaaatattatttcccttctgagacagtcctgcagcctgtgcctccactttacaccaacagaagcttgtgttcaggccttgccctctggaagattacaaattaatggagacaggataaacacatggaaaaatacctagagggaaaaaaagatataagaggcttataaacagagccaattaaagttatacagttatttacatgatcgctgagaggcttctgcttgagtagaggacggggtgagcagagtcccatcctgggggtgagttctcagtgggatattgaaggagagaaagttcacgatttggcagtggtggaagtacagcattctagaggagggaaataacttgaaggtgagagcaagtgaactgtgtgtgatggtttttccaccg

SEQ ID NO: 9715 - RNA, 6406 nt, Homo sapiens
  source 1..6406: mol_type = other RNA
atgcacctgggcaaggattctgatagagaagaattttggctcatctctgaaaaaacattttcacatagaaattccttctctgggtttggcaaagcattctgatgacctttttgtaatgttggcacagaattttgttcttcactgattggcactacactatgattagtctggcaaattggctgattgggcagatcttgggtcactagtatttgtggcagggatgtgagtgtagcaaaacagtaagcaggaacactactctgcaggcgtatgggcagcatgaatgatgatggcaccttctgcacctgacttccaaggggcctgagctctggtggtagcagaggatgcgaattagacatgctgtcaattaatttggttggtaatgttgctgatgtcacacaatgatctgttccaactggatctgaaataacttgatttggcaaagaatgcacaggattagaagagcaagatgggcctgaagtgaaaacctgacaatgcaattggtatttgggagcaaagcaatcctcacttttagaagacccagataaaacagaatttttatctggcttgctaccctgcgtagacacttgcagagatagctgtgtgctctggtggctaggcggtgcatggatttgatttaacaaattgatatcacagagctgttgaacaggaaaaacgttggtagagctggagtttgatgtttctgcctgcagatccttaacctgagtctgagagtgcaaagtatttgcagaaaactcagctaaagatgtactagtgagctgaggcccctgatatggcactgcattcacactgggaagagcagtattttggaaagatgttgggtgtacaggagacagatgactatctggggctatgtttaaagatatttgccgtaccagtgggcctctccttctttctaagagaggcacatgcccagtcactcccactcgagaaggtgaagatggaggctgcaattcagtaagtggtgttgtctggggtggggtgatgcttccacaatcgaatgatttgcttctgagatcagagacctccattgacgtttgcgtgcaattaatctgttctgatgcagtacgcctcatttcccggtgacatccaggaacattcagagtattcaagccagctggaatcataagaaactcggctttatttagaaaatcgattttgggggaagcctccgttttagaaacgtcctctatgtctaaagaggctgagaaacttgaagtgtgagataaactgctctccctacttagactcctggagagagtggaatcaaagctcgattctgttgaggaatgttctatctcagccagacggagccttttctttttgggtggcagtttctctgttggcaattttgacaaggtttcactacgctggggccaactgaacttctctgacttttcttgatcatggcattgagcttccaggtctcgatctggttcttctgtgaccaaaatctctggaacttggatgttgtgctgccggacaagtcttgagggctgtcctaacacatgtcgttcacttggactctttctggagctttcctgaagttctcctctgagagcgtctgatagtgcaagctggtgaggatgagacccgtcccgagaagggtgactttcctcttgggagattcctatcacttttagagacccggacttccccgttctattcagctcctggaaagaaactggggaggctctttcaaaaggctcaggcttgtcaaatgagttgggcctgctcagggagttggtgtgctggatgacagagattccagttccgtgtctctgcagttctatcttgtcctgggctgctgaacttatctgttgttccatgatggtcgacagcttgggatccatggtctgctcagggcccctggcaacaaggtgaatatgggagttttgcaactgtatatttttatgctgctggtcacttcttatggtaacattatgtttaggcaaactgggattacagcccagagcattctgaaactgaaggccttcagaactttttggagatgttccactttcattttgctgaagttcttcatcatccccaacacttttcattttcctcctttttcttatctggggcgtctgttcccagatgccggaggacccagcgactctgtagtgtagaatctgaggctgcagaccgccgggcacagggctgtgctcaggttctctcatggctacctttgtttttggtccatgtaactcagaacagtaaaatttcttatgattttcaaaattttccagtttcctatacctgtttctacaagtttcacactcaaacattgtccctcgcccttgatgagacttctttttttctatatgtgggccttgtgccagtgccttgctcctcactgacatggcttcaccagcagcatggcatccttggtggctctcatccagggactgtccagtaccaagaacatgactttcatttgctgaagagtcttctatggctgcttgtctcacaagtgtacggggatgcccactctggggcacaggagcgttaggtcccgatacaaagacatcatcatagaaagcgccaattttgtcatcaaatgactgacttcctcttagtggatgaggaggaggtattatatttgcaggtactgctgaataacctgtggtcggcatggaattacttcttgtgataggtaaacagtcaagtgaaggtacagacagaagaaacacttgctttgatttttcagtaggggtgaaaggtgacttcggtatatcagagcttgaacttgttctccgtcccactggttttaaatcaaactggaaagaatctttaaatatgtatgatttgggggaatcaatgcttcctcgtcttgacagtgaggttctccgcggcttcacactatccagttgcttgtcatctaccaaagcttcattgtctgagataagcttcgatatccgctcctcaagtgtttttgtggccaaaggtgggcgcatctgacctggtaaaagcaatgccttttcccctgtgggcaaagcagagggtgttgacgtggtgacaagagctgcagagggtccgttactccttccagagtcttgttctgtgctgggtaaccttctggcaaagggagttggtggactcactgtttgatcggcactttcagaacgtgaaaagtaaccagaatccgtacttcctaaacttcgaggactcaggagctttccttgctgctcttgggagtaatcggtagcctgctgcctttgtagctgggcgtgtaccgttcctacgtgagagtcttgctttccttccagtggattcatgtcgcctttctggtgggaattctcattagtctccaacctggagactccaccctgggacatgttggctgaaagtggctgtacgtttgtcacctgaaggtccttctgcttttgtgcactagaaagttcaggcttgggatccatggcctttggactgtcagttcttaagggggacacagtgacatggtggaccacaactttcggtaactctgtcacagcttgtgattctgcagatctgtcctgtagcaaaaagtcacctatcacattttctggactgcttggagtgaagcttgattttagtaaagtttcagcatttgacatcctctttattatgtgcacaggctgcagctccatggcgcccaggtcatgctgtctctcatcagtggcgccttcctcctcgctctccccactgtcttctacgtctgaatgaatactaagtgctttgggggactcgtgggacaagaacaagccaccagcatctggttgcaagacaagacccagtttgatagtatgtgcgtgggatttcttgtgcttatacagattacttttagtcttaaatgaaaatccacaagtcacacagggatagggtcgctctccagtgtgggagcggatatgctttaaaagcacactaggctttgcacatgctctattgcaatactcacaaatatattttccttgtttttttggcttctgatctttcagaagaagattgcacatttgctctacgctttgattaacaacagaggcaacatgagttgaattatagattggcatggggggcgactgtgtagaattagccggacttattgacaaaggtgaagcagaatccatttgctggttttgaggagtaacctgagatctactggaaggtgaagttaggcctacagatgatgtcactgctatattataaacctgttcaagtttggcattctcttgattttgcagatttgtcagtgatcctgtgaaacctgaacaccccggaagctgttgattatgttggttggatttgggaacaaagtgttcatgttgatgatacaaatgagaagctgactgcattgccccttgctcattcttctgagcagcagacatatggactgtgtatgaggtacaagaagactgtgattcagcaaccaattcctgtgaagtctgatttggggcatccattgaactgttttttaatttgggaggggaacgtgcagttttatttggcctcagtttttctgtcttaattgcacaaggtgagcccttttgtgacaaggtgctcagttctggctccattgctttcagtaagacatcgaatgcagtgtttgtataggagggggacgtagtgccacaatgagaagagatgcattcgctattgtcagtcctggttttacttgacaaggaacttgagtcacattgttcatcgaggtcactgaatttggcaggatcagcgccttcggatctccatctacgcagttcagatggttgctgcagaaacaagggcttctttggggagacagattcttcagattttgaggcttcagcaattattccaggtgtttctccattttgtttggtaaactgcttcccattttttacaggaatataattctgtttcttgtgagactccgaagcactatgaagaacggcgaaagatgactcttctgtattttgtttatgttttgcctgaagaggatttctcagtggggattttggtatttttttcaggtgattctcagctacgatctttttgcgtttcacacctttaagggattccgaagttcctttaacaccagcctgtaagatttctttttttgaaacttctgccccattaagttctttttgtgcttcttcaattttgtcaagaccatgcggaagagccaccccgtgcagtccagtgacccttctccacggaacccaggacaacatgctaagcctttcttctgaacaccaagtgctgctctcatgctcttccaaaattcttcaacctcacaaaggataggtcggtgtcaaaacggcacccaccacgtttcctcttagatttctgggatgaatttgtttagttcgaggcatcttctttgactcagggccttctttttcttcttaaaaactgcagataaagcaagccaccaaaaggcagctccataaactcaacatacatcaattaatccatgtgccgaactgcaacacaaaagtctgatccaaagcttcctgggtttaacttttaattttaaaaacaaaaaagcagaaaccaaaagcctcctaggttggaagtgggcgtgagaggaaatgctagagggaggcgcttcattccccgggctgcctgtgcccccctttctggcccctgcccggggctttgatgttatctagtgcaccgcctccatcggtttctaccttgggctctgcgccgccgagaagatagacagatcttccgcacttcacttgcaggttctgagagaggcaagcaggtagtcgcgggaaaggacccacactccttagccccgcagtgagagaggaacatttgcacgggcttcctgttgctacctggactgaaatgaacaatccacccctctagtgatcctggagacttgcaccgtatggtctttcctgctagacgcacagcgggaggcctcctacattagattcattttccctccacccgtagcacaaacttgtaagatggtggtggagtatgtttcctgaggctttgttcgggttttagatctcagtttggaaggtaaatattatttcccttctgagacagtcctgcagcctgtgcctccactttacaccaacagaagcttgtgttcaggccttgccctctggaagattacaaattaatggagacaggataaacacatggaaaaatacctagagggaaaaaaagatataagaggcttataaacagagccaattaaagttatacagttatttacatgatcgctgagaggcttctgcttgagtagaggacggggtgagcagagtcccatcctgggggtgagttctcagtgggatattgaaggagagaaagttcacgatttggcagtggtggaagtacagcattctagaggagggaaataacttgaaggtgagagcaagtgaactgtgtgtgatggtttttccaccga

SEQ ID NO: 9716 - RNA, 6308 nt, Homo sapiens
  source 1..6308: mol_type = other RNA
atgcacctgggcaaggattctgatagagaagaattttggctcatctctgaaaaaacattttcacatagaaattccttctctgggtttggcaaagcattctgatgacctttttgtaatgttggcacagaattttgttcttcactgattggcactacactatgattagtctggcaaattggctgattgggcagatcttgggtcactagtatttgtggcagggatgtgagtgtagcaaaacagtaagcaggaacactactctgcaggcgtatgggcagcatgaatgatgatggcaccttctgcacctgacttccaaggggcctgagctctggtggtagcagaggatgcgaattagacatgctgtcaattaatttggttggtaatgttgctgatgtcacacaatgatctgttccaactggatctgaaataacttgatttggcaaagaatgcacaggattagaagagcaagatgggcctgaagtgaaaacctgacaatgcaattggtatttgggagcaaagcaatcctcacttttagaagacccagataaaacagaatttttatctggcttgctaccctgcgtagacacttgcagagatagctgtgtgctctggtggctaggcggtgcatggatttgatttaacaaattgatatcacagagctgttgaacaggaaaaacgttggtagagctggagtttgatgtttctgcctgcagatccttaacctgagtctgagagtgcaaagtatttgcagaaaactcagctaaagatgtactagtgagctgaggcccctgatatggcactgcattcacactgggaagagcagtattttggaaagatgttgggtgtacaggagacagatgactatctggggctatgtttaaagatatttgccgtaccagtgggcctctccttctttctaagagaggcacatgcccagtcactcccactcgagaaggtgaagatggaggctgcaattcagtaagtggtgttgtctggggtggggtgatgcttccacaatcgaatgatttgcttctgagatcagagacctccattgacgtttgcgtgcaattaatctgttctgatgcagtacgcctcatttcccggtgacatccaggaacattcagagtattcaagccagctggaatcataagaaactcggctttatttagaaaatcgattttgggggaagcctccgttttagaaacgtcctctatgtctaaagaggctgagaaacttgaagtgtgagataaactgctctccctacttagactcctggagagagtggaatcaaagctcgattctgttgaggaatgttctatctcagccagacggagccttttctttttgggtggcagtttctctgttggcaattttgacaaggtttcactacgctggggccaactgaacttctctgacttttcttgatcatggcattgagcttccaggtctcgatctggttcttctgtgaccaaaatctctggaacttggatgttgtgctgccggacaagtcttgagggctgtcctaacacatgtcgttcacttggactctttctggagctttcctgaagttctcctctgagagcgtctgatagtgcaagctggtgaggatgagacccgtcccgagaagggtgactttcctcttgggagattcctatcacttttagagacccggacttccccgttctattcagctcctggaaagaaactggggaggctctttcaaaaggctcaggcttgtcaaatgagttgggcctgctcagggagttggtgtgctggatgacagagattccagttccgtgtctctgcagttctatcttgtcctgggctgctgaacttatctgttgttccatgatggtcgacagcttgggatccatggtctgctcagggcccctggcaacaaggtgaatatgggagttttgcaactgtatatttttatgctgctggtcacttcttatggtaacattatgtttaggcaaactgggattacagcccagagcattctgaaactgaaggccttcagaactttttggagatgttccactttcattttgctgaagttcttcatcatccccaacacttttcattttcctcctttttcttatctggggcgtctgttcccagatgccggaggacccagcgactctgtagtgtagaatctgaggctgcagaccgccgggcacagggctgtgctcaggttctctcatggctacctttgtttttggtccatgtaactcagaacagtaaaatttcttatgattttcaaaattttccagtttcctatacctgtttctacaagtttcacactcaaacattgtccctcgcccttgatgagacttctttttttctatatgtgggccttgtgccagtgccttgctcctcactgacatggcttcaccagcagcatggcatccttggtggctctcatccagggactgtccagtaccaagaacatgactttcatttgctgaagagtcttctatggctgcttgtctcacaagtgtacggggatgcccactctggggcacaggagcgttaggtcccgatacaaagacatcatcatagaaagcgccaattttgtcatcaaatgactgacttcctcttagtggatgaggaggaggtattatatttgcaggtactgctgaataacctgtggtcggcatggaattacttcttgtgataggtaaacagtcaagtgaaggtacagacagaagaaacacttgctttgatttttcagtaggggtgaaaggtgacttcggtatatcagagcttgaacttgttctccgtcccactggttttaaatcaaactggaaagaatctttaaatatgtatgatttgggggaatcaatgcttcctcgtcttgacagtgaggttctccgcggcttcacactatccagttgcttgtcatctaccaaagcttcattgtctgagataagcttcgatatccgctcctcaagtgtttttgtggccaaaggtgggcgcatctgacctggtaaaagcaatgccttttcccctgtgggcaaagcagagggtgttgacgtggtgacaagagctgcagagggtccgttactccttccagagtcttgttctgtgctgggtaaccttctggcaaagggagttggtggactcactgtttgatcggcactttcagaacgtgaaaagtaaccagaatccgtacttcctaaacttcgaggactcaggagctttccttgctgctcttgggagtaatcggtagcctgctgcctttgtagctgggcgtgtaccgttcctacgtgagagtcttgctttccttccagtggattcatgtcgcctttctggtgggaattctcattagtctccaacctggagactccaccctgggacatgttggctgaaagtggctgtacgtttgtcacctgaaggtccttctgcttttgtgcactagaaagttcaggcttgggatccatggcctttggactgtcagttcttaagggggacacagtgacatggtggaccacaactttcggtaactctgtcacagcttgtgattctgcagatctgtcctgtagcaaaaagtcacctatcacattttctggactgcttggagtgaagcttgattttagtaaagtttcagcatttgacatcctctttattatgtgcacaggctgcagctccatggcgcccaggtcatgctgtctctcatcagtggcgccttcctcctcgctctccccactgtcttctacgtctgaatgaatactaagtgctttgggggactcgtgggacaagaacaagccaccagcatctggttgcaagacaagacccagtttgatagtatgtgcgtgggatttcttgtgcttatacagattacttttagtcttaaatgaaaatccacaagtcacacagggatagggtcgctctccagtgtgggagcggatatgctttaaaagcacactaggctttgcacatgctctattgcaatactcacaaatatattttccttgtttttttggcttctgatctttcagaagaagattgcacatttgctctacgctttgattaacaacagaggcaacatgagttgaattatagattggcatggggggcgactgtgtagaattagccggacttattgacaaaggtgaagcagaatccatttgctggttttgaggagtaacctgagatctactggaaggtgaagttaggcctacagatgatgtcactgctatattataaacctgttcaagtttggcattctcttgattttgcagatttgtcagtgatcctgtgaaacctgaacaccccggaagctgttgattatgttggttggatttgggaacaaagtgttcatgttgatgatacaaatgagaagctgactgcattgccccttgctcattcttctgagcagcagacatatggactgtgtatgaggtacaagaagactgtgattcagcaaccaattcctgtgaagtctgatttggggcatccattgaactgttttttaatttgggaggggaacgtgcagttttatttggcctcagtttttctgtcttaattgcacaaggtgagcccttttgtgacaaggtgctcagttctggctccattgctttcagtaagacatcgaatgcagtgtttgtataggagggggacgtagtgccacaatgagaagagatgcattcgctattgtcagtcctggttttacttgacaaggaacttgagtcacattgttcatcgaggtcactgaatttggcaggatcagcgccttcggatctccatctacgcagttcagatggttgctgcagaaacaagggcttctttggggagacagattcttcagattttgaggcttcagcaattattccaggtgtttctccattttgtttggtaaactgcttcccattttttacaggaatataattctgtttcttgtgagactccgaagcactatgaagaacggcgaaagatgactcttctgtattttgtttatgttttgcctgaagaggatttctcagtggggattttggtatttttttcaggtgattctcagctacgatctttttgcgtttcacacctttaagggattccgaagttcctttaacaccagcctgtaagatttctttttttgaaacttctgccccattaagttctttttgtgcttcttcaattttgtcaagaccatgcggaagagccaccccgtgcagtccagtgacccttctccacggaacccaggacaacatgctaagcctttcttctgaacaccaagtgctgctctcatgctcttccaaaattcttcaacctcacaaaggataggtcggtgtcaaaacggcacccaccacgtttcctcttagatttctgggatgaatttgtttagttcgaggcatcttctttgactcagggccttctttttcttcttaaaaactgcagataaagcaagccaccaaaaggcagctccataaactcaacatacatcaattaatccatgtgccgaactgcaacacaaaagtctgatccaaagcttcctgggtttaacttttaattttaaaaacaaaaaagcagaaaccaaaagcctcctaggttggaagtgggcgtgagaggaaatgctagagggaggcgcttcattccccgggctgcctgtgcccccctttctggcccctgcccggggctttgatgttatctagtgcaccgcctccatcggtttctaccttgggctctgcgccgccgagaagatagacagatcttccgcacttcacttgcaggttctgagagaggcaagcaggtagtcgcgggaaaggacccacactccttagccccgcagtgagagaggaacatttgcacgggcttcctgttgctacctggactgaaatgaacaatccacccctctagtgatcctggagacttgcaccgtatggtctttcctgctagacgcacagcgggaggcctcctacattagattcattttccctccacccgtagcacaaacttgtaagatggtggtggagtatgtttcctgaggctttgttcgggttttagatctcagtttggaaggtaaatattatttcccttctgagacagtcctgcagccttgaaaagacaagaataaaaatctaaaggcaacaaattctataacatgctttccatacaccataaattcccttatgggtcaaaatatccgcacactttcccctcacgttatgaaaagcttgtaactgttgattttcttttgtctggacactagcagacactggatatagtttttcattaggttagcagtctcgggaccatcactaacaaaacactacaacaaagaatttttttttttttaacagattactaataaa

SEQ ID NO: 9717 - RNA, 5561 nt, Homo sapiens
  source 1..5561: mol_type = other RNA
atgcacctgggcaaggattctgatagagaagaattttggctcatctctgaaaaaacattttcacatagaaattccttctctgggtttggcaaagcattctgatgacctttttgtaatgttggcacagaattttgttcttcactgattggcactacactatgattagtctggcaaattggctgattgggcagatcttgggtcactagtatttgtggcagggatgtgagtgtagcaaaacagtaagcaggaacactactctgcaggcgtatgggcagcatgaatgatgatggcaccttctgcacctgacttccaaggggcctgagctctggtggtagcagaggatgcgaattagacatgctgtcaattaatttggttggtaatgttgctgatgtcacacaatgatctgttccaactggatctgaaataacttgatttggcaaagaatgcacaggattagaagagcaagatgggcctgaagtgaaaacctgacaatgcaattggtatttgggagcaaagcaatcctcacttttagaagacccagataaaacagaatttttatctggcttgctaccctgcgtagacacttgcagagatagctgtgtgctctggtggctaggcggtgcatggatttgatttaacaaattgatatcacagagctgttgaacaggaaaaacgttggtagagctggagtttgatgtttctgcctgcagatccttaacctgagtctgagagtgcaaagtatttgcagaaaactcagctaaagatgtactagtgagctgaggcccctgatatggcactgcattcacactgggaagagcagtattttggaaagatgttgggtgtacaggagacagatgactatctggggctatgtttaaagatatttgccgtaccagtgggcctctccttctttctaagagaggcacatgcccagtcactcccactcgagaaggtgaagatggaggctgcaattcagtaagtggtgttgtctggggtggggtgatgcttccacaatcgaatgatttgcttctgagatcagagacctccattgacgtttgcgtgcaattaatctgttctgatgcagtacgcctcatttcccggtgacatccaggaacattcagagtattcaagccagctggaatcataagaaactcggctttatttagaaaatcgattttgggggaagcctccgttttagaaacgtcctctatgtctaaagaggctgagaaacttgaagtgtgagataaactgctctccctacttagactcctggagagagtggaatcaaagctcgattctgttgaggaatgttctatctcagccagacggagccttttctttttgggtggcagtttctctgttggcaattttgacaaggtttcactacgctggggccaactgaacttctctgacttttcttgatcatggcattgagcttccaggtctcgatctggttcttctgtgaccaaaatctctggaacttggatgttgtgctgccggacaagtcttgagggctgtcctaacacatgtcgttcacttggactctttctggagctttcctgaagttctcctctgagagcgtctgatagtgcaagctggtgaggatgagacccgtcccgagaagggtgactttcctcttgggagattcctatcacttttagagacccggacttccccgttctattcagctcctggaaagaaactggggaggctctttcaaaaggctcaggcttgtcaaatgagttgggcctgctcagggagttggtgtgctggatgacagagattccagttccgtgtctctgcagttctatcttgtcctgggctgctgaacttatctgttgttccatgatggtcgacagcttgggatccatggtctgctcagggcccctggcaacaaggtgaatatgggagttttgcaactgtatatttttatgctgctggtcacttcttatggtaacattatgtttaggcaaactgggattacagcccagagcattctgaaactgaaggccttcagaactttttggagatgttccactttcattttgctgaagttcttcatcatccccaacacttttcattttcctcctttttcttatctggggcgtctgttcccagatgccggaggacccagcgactctgtagtgtagaatctgaggctgcagaccgccgggcacagggctgtgctcaggttctctcatggctacctttgtttttggtccatgtaactcagaacagtaaaatttcttatgattttcaaaattttccagtttcctatacctgtttctacaagtttcacactcaaacattgtccctcgcccttgatgagacttctttttttctatatgtgggccttgtgccagtgccttgctcctcactgacatggcttcaccagcagcatggcatccttggtggctctcatccagggactgtccagtaccaagaacatgactttcatttgctgaagagtcttctatggctgcttgtctcacaagtgtacggggatgcccactctggggcacaggagcgttaggtcccgatacaaagacatcatcatagaaagcgccaattttgtcatcaaatgactgacttcctcttagtggatgaggaggaggtattatatttgcaggtactgctgaataacctgtggtcggcatggaattacttcttgtgataggtaaacagtcaagtgaaggtacagacagaagaaacacttgctttgatttttcagtaggggtgaaaggtgacttcggtatatcagagcttgaacttgttctccgtcccactggttttaaatcaaactggaaagaatctttaaatatgtatgatttgggggaatcaatgcttcctcgtcttgacagtgaggttctccgcggcttcacactatccagttgcttgtcatctaccaaagcttcattgtctgagataagcttcgatatccgctcctcaagtgtttttgtggccaaaggtgggcgcatctgacctggtaaaagcaatgccttttcccctgtgggcaaagcagagggtgttgacgtggtgacaagagctgcagagggtccgttactccttccagagtcttgttctgtgctgggtaaccttctggcaaagggagttggtggactcactgtttgatcggcactttcagaacgtgaaaagtaaccagaatccgtacttcctaaacttcgaggactcaggagctttccttgctgctcttgggagtaatcggtagcctgctgcctttgtagctgggcgtgtaccgttcctacgtgagagtcttgctttccttccagtggattcatgtcgcctttctggtgggaattctcattagtctccaacctggagactccaccctgggacatgttggctgaaagtggctgtacgtttgtcacctgaaggtccttctgcttttgtgcactagaaagttcaggcttgggatccatggcctttggactgtcagttcttaagggggacacagtgacatggtggaccacaactttcggtaactctgtcacagcttgtgattctgcagatctgtcctgtagcaaaaagtcacctatcacattttctggactgcttggagtgaagcttgattttagtaaagtttcagcatttgacatcctctttattatgtgcacaggctgcagctccatggcgcccaggtcatgctgtctctcatcagtggcgccttcctcctcgctctccccactgtcttctacgtctgaatgaatactaagtgctttgggggactcgtgggacaagaacaagccaccagcatctggttgcaagacaagacccagtttgatagtatgtgcgtgggatttcttgtgcttatacagattacttttagtcttaaatgaaaatccacaagtcacacagggatagggtcgctctccagtgtgggagcggatatgctttaaaagcacactaggctttgcacatgctctattgcaatactcacaaatatattttccttgtttttttggcttctgatctttcagaagaagattgcacatttgctctacgctttgattaacaacagaggcaacatgagttgaattatagattggcatggggggcgactgtgtagaattagccggacttattgacaaaggtgaagcagaatccatttgctggttttgaggagtaacctgagatctactggaaggtgaagttaggcctacagatgatgtcactgctatattataaacctgttcaagtttggcattctcttgattttgcagatttgtcagtgatcctgtgaaacctgaacaccccggaagctgttgattatgttggttggatttgggaacaaagtgttcatgttgatgatacaaatgagaagctgactgcattgccccttgctcattcttctgagcagcagacatatggactgtgtatgaggtacaagaagactgtgattcagcaaccaattcctgtgaagtctgatttggggcatccattgaactgttttttaatttgggaggggaacgtgcagttttatttggcctcagtttttctgtcttaattgcacaaggtgagcccttttgtgacaaggtgctcagttctggctccattgctttcagtaagacatcgaatgcagtgtttgtataggagggggacgtagtgccacaatgagaagagatgcattcgctattgtcagtcctggttttacttgacaaggaacttgagtcacattgttcatcgaggtcactgaatttggcaggatcagcgccttcggatctccatctacgcagttcagatggttgctgcagaaacaagggcttctttggggagacagattcttcagattttgaggcttcagcaattattccaggtgtttctccattttgtttggtaaactgcttcccattttttacaggaatataattctgtttcttgtgagactccgaagcactatgaagaacggcgaaagatgactcttctgtattttgtttatgttttgcctgaagaggatttctcagtggggattttggtatttttttcaggtgattctcagctacgatctttttgcgtttcacacctttaagggattccgaagttcctttaacaccagcctgtaagatttctttttttgaaacttctgccccattaagttctttttgtgcttcttcaattttgtcaagaccatgcggaagagccaccccgtgcagtccagtgacccttctccacggaacccaggacaacatgctaagcctttcttctgaacaccaagtgctgctctcatgctcttccaaaattcttcaacctcacaaaggataggtcggtgtcaaaacggcacccaccacgtttcctcttagatttctgggatgaatttgtttagttcgaggcatcttctttgactcagggccttctttttcttcttaaaaactgcagataaagcaagccaccaaaaggcagctccataaactcaacatacatcaattaatccatgtgctctcccccggggcagagtagggcacgtttagcgtctttggggccggcgggaggaacgcgggccgggcggcgcgggggaggcagggcgaaggtcggaggctttcccg

SEQ ID NO: 9718 - RNA, 5552 nt, Homo sapiens
  source 1..5552: mol_type = other RNA
atgcacctgggcaaggattctgatagagaagaattttggctcatctctgaaaaaacattttcacatagaaattccttctctgggtttggcaaagcattctgatgacctttttgtaatgttggcacagaattttgttcttcactgattggcactacactatgattagtctggcaaattggctgattgggcagatcttgggtcactagtatttgtggcagggatgtgagtgtagcaaaacagtaagcaggaacactactctgcaggcgtatgggcagcatgaatgatgatggcaccttctgcacctgacttccaaggggcctgagctctggtggtagcagaggatgcgaattagacatgctgtcaattaatttggttggtaatgttgctgatgtcacacaatgatctgttccaactggatctgaaataacttgatttggcaaagaatgcacaggattagaagagcaagatgggcctgaagtgaaaacctgacaatgcaattggtatttgggagcaaagcaatcctcacttttagaagacccagataaaacagaatttttatctggcttgctaccctgcgtagacacttgcagagatagctgtgtgctctggtggctaggcggtgcatggatttgatttaacaaattgatatcacagagctgttgaacaggaaaaacgttggtagagctggagtttgatgtttctgcctgcagatccttaacctgagtctgagagtgcaaagtatttgcagaaaactcagctaaagatgtactagtgagctgaggcccctgatatggcactgcattcacactgggaagagcagtattttggaaagatgttgggtgtacaggagacagatgactatctggggctatgtttaaagatatttgccgtaccagtgggcctctccttctttctaagagaggcacatgcccagtcactcccactcgagaaggtgaagatggaggctgcaattcagtaagtggtgttgtctggggtggggtgatgcttccacaatcgaatgatttgcttctgagatcagagacctccattgacgtttgcgtgcaattaatctgttctgatgcagtacgcctcatttcccggtgacatccaggaacattcagagtattcaagccagctggaatcataagaaactcggctttatttagaaaatcgattttgggggaagcctccgttttagaaacgtcctctatgtctaaagaggctgagaaacttgaagtgtgagataaactgctctccctacttagactcctggagagagtggaatcaaagctcgattctgttgaggaatgttctatctcagccagacggagccttttctttttgggtggcagtttctctgttggcaattttgacaaggtttcactacgctggggccaactgaacttctctgacttttcttgatcatggcattgagcttccaggtctcgatctggttcttctgtgaccaaaatctctggaacttggatgttgtgctgccggacaagtcttgagggctgtcctaacacatgtcgttcacttggactctttctggagctttcctgaagttctcctctgagagcgtctgatagtgcaagctggtgaggatgagacccgtcccgagaagggtgactttcctcttgggagattcctatcacttttagagacccggacttccccgttctattcagctcctggaaagaaactggggaggctctttcaaaaggctcaggcttgtcaaatgagttgggcctgctcagggagttggtgtgctggatgacagagattccagttccgtgtctctgcagttctatcttgtcctgggctgctgaacttatctgttgttccatgatggtcgacagcttgggatccatggtctgctcagggcccctggcaacaaggtgaatatgggagttttgcaactgtatatttttatgctgctggtcacttcttatggtaacattatgtttaggcaaactgggattacagcccagagcattctgaaactgaaggccttcagaactttttggagatgttccactttcattttgctgaagttcttcatcatccccaacacttttcattttcctcctttttcttatctggggcgtctgttcccagatgccggaggacccagcgactctgtagtgtagaatctgaggctgcagaccgccgggcacagggctgtgctcaggttctctcatggctacctttgtttttggtccatgtaactcagaacagtaaaatttcttatgattttcaaaattttccagtttcctatacctgtttctacaagtttcacactcaaacattgtccctcgcccttgatgagacttctttttttctatatgtgggccttgtgccagtgccttgctcctcactgacatggcttcaccagcagcatggcatccttggtggctctcatccagggactgtccagtaccaagaacatgactttcatttgctgaagagtcttctatggctgcttgtctcacaagtgtacggggatgcccactctggggcacaggagcgttaggtcccgatacaaagacatcatcatagaaagcgccaattttgtcatcaaatgactgacttcctcttagtggatgaggaggaggtattatatttgcaggtactgctgaataacctgtggtcggcatggaattacttcttgtgataggtaaacagtcaagtgaaggtacagacagaagaaacacttgctttgatttttcagtaggggtgaaaggtgacttcggtatatcagagcttgaacttgttctccgtcccactggttttaaatcaaactggaaagaatctttaaatatgtatgatttgggggaatcaatgcttcctcgtcttgacagtgaggttctccgcggcttcacactatccagttgcttgtcatctaccaaagcttcattgtctgagataagcttcgatatccgctcctcaagtgtttttgtggccaaaggtgggcgcatctgacctggtaaaagcaatgccttttcccctgtgggcaaagcagagggtgttgacgtggtgacaagagctgcagagggtccgttactccttccagagtcttgttctgtgctgggtaaccttctggcaaagggagttggtggactcactgtttgatcggcactttcagaacgtgaaaagtaaccagaatccgtacttcctaaacttcgaggactcaggagctttccttgctgctcttgggagtaatcggtagcctgctgcctttgtagctgggcgtgtaccgttcctacgtgagagtcttgctttccttccagtggattcatgtcgcctttctggtgggaattctcattagtctccaacctggagactccaccctgggacatgttggctgaaagtggctgtacgtttgtcacctgaaggtccttctgcttttgtgcactagaaagttcaggcttgggatccatggcctttggactgtcagttcttaagggggacacagtgacatggtggaccacaactttcggtaactctgtcacagcttgtgattctgcagatctgtcctgtagcaaaaagtcacctatcacattttctggactgcttggagtgaagcttgattttagtaaagtttcagcatttgacatcctctttattatgtgcacaggctgcagctccatggcgcccaggtcatgctgtctctcatcagtggcgccttcctcctcgctctccccactgtcttctacgtctgaatgaatactaagtgctttgggggactcgtgggacaagaacaagccaccagcatctggttgcaagacaagacccagtttgatagtatgtgcgtgggatttcttgtgcttatacagattacttttagtcttaaatgaaaatccacaagtcacacagggatagggtcgctctccagtgtgggagcggatatgctttaaaagcacactaggctttgcacatgctctattgcaatactcacaaatatattttccttgtttttttggcttctgatctttcagaagaagattgcacatttgctctacgctttgattaacaacagaggcaacatgagttgaattatagattggcatggggggcgactgtgtagaattagccggacttattgacaaaggtgaagcagaatccatttgctggttttgaggagtaacctgagatctactggaaggtgaagttaggcctacagatgatgtcactgctatattataaacctgttcaagtttggcattctcttgattttgcagatttgtcagtgatcctgtgaaacctgaacaccccggaagctgttgattatgttggttggatttgggaacaaagtgttcatgttgatgatacaaatgagaagctgactgcattgccccttgctcattcttctgagcagcagacatatggactgtgtatgaggtacaagaagactgtgattcagcaaccaattcctgtgaagtctgatttggggcatccattgaactgttttttaatttgggaggggaacgtgcagttttatttggcctcagtttttctgtcttaattgcacaaggtgagcccttttgtgacaaggtgctcagttctggctccattgctttcagtaagacatcgaatgcagtgtttgtataggagggggacgtagtgccacaatgagaagagatgcattcgctattgtcagtcctggttttacttgacaaggaacttgagtcacattgttcatcgaggtcactgaatttggcaggatcagcgccttcggatctccatctacgcagttcagatggttgctgcagaaacaagggcttctttggggagacagattcttcagattttgaggcttcagcaattattccaggtgtttctccattttgtttggtaaactgcttcccattttttacaggaatataattctgtttcttgtgagactccgaagcactatgaagaacggcgaaagatgactcttctgtattttgtttatgttttgcctgaagaggatttctcagtggggattttggtatttttttcaggtgattctcagctacgatctttttgcgtttcacacctttaagggattccgaagttcctttaacaccagcctgtaagatttctttttttgaaacttctgccccattaagttctttttgtgcttcttcaattttgtcaagaccatgcggaagagccaccccgtgcagtccagtgacccttctccacggaacccaggacaacatgctaagcctttcttctgaacaccaagtgctgctctcatgctcttccaaaattcttcaacctcacaaaggataggtcggtgtcaaaacggcacccaccacgtttcctcttagatttctgggatgaatttgtttagttcgaggcatcttctttgactcagggccttctttttcttcttaaaaactgcagataaagcaagccaccaaaaggcagctccataaactcaacatacatcaattaatccatgtgctgctcggctcgcgcgcggcgagggcgcccagaagtgccaagggtctcccgcacgcagccatcccctctgcaaggtcggcggttgcacacacacgcac

SEQ ID NO: 9719 - RNA, 5686 nt, Homo sapiens
  source 1..5686: mol_type = other RNA
atgcacctgggcaaggattctgatagagaagaattttggctcatctctgaaaaaacattttcacatagaaattccttctctgggtttggcaaagcattctgatgacctttttgtaatgttggcacagaattttgttcttcactgattggcactacactatgattagtctggcaaattggctgattgggcagatcttgggtcactagtatttgtggcagggatgtgagtgtagcaaaacagtaagcaggaacactactctgcaggcgtatgggcagcatgaatgatgatggcaccttctgcacctgacttccaaggggcctgagctctggtggtagcagaggatgcgaattagacatgctgtcaattaatttggttggtaatgttgctgatgtcacacaatgatctgttccaactggatctgaaataacttgatttggcaaagaatgcacaggattagaagagcaagatgggcctgaagtgaaaacctgacaatgcaattggtatttgggagcaaagcaatcctcacttttagaagacccagataaaacagaatttttatctggcttgctaccctgcgtagacacttgcagagatagctgtgtgctctggtggctaggcggtgcatggatttgatttaacaaattgatatcacagagctgttgaacaggaaaaacgttggtagagctggagtttgatgtttctgcctgcagatccttaacctgagtctgagagtgcaaagtatttgcagaaaactcagctaaagatgtactagtgagctgaggcccctgatatggcactgcattcacactgggaagagcagtattttggaaagatgttgggtgtacaggagacagatgactatctggggctatgtttaaagatatttgccgtaccagtgggcctctccttctttctaagagaggcacatgcccagtcactcccactcgagaaggtgaagatggaggctgcaattcagtaagtggtgttgtctggggtggggtgatgcttccacaatcgaatgatttgcttctgagatcagagacctccattgacgtttgcgtgcaattaatctgttctgatgcagtacgcctcatttcccggtgacatccaggaacattcagagtattcaagccagctggaatcataagaaactcggctttatttagaaaatcgattttgggggaagcctccgttttagaaacgtcctctatgtctaaagaggctgagaaacttgaagtgtgagataaactgctctccctacttagactcctggagagagtggaatcaaagctcgattctgttgaggaatgttctatctcagccagacggagccttttctttttgggtggcagtttctctgttggcaattttgacaaggtttcactacgctggggccaactgaacttctctgacttttcttgatcatggcattgagcttccaggtctcgatctggttcttctgtgaccaaaatctctggaacttggatgttgtgctgccggacaagtcttgagggctgtcctaacacatgtcgttcacttggactctttctggagctttcctgaagttctcctctgagagcgtctgatagtgcaagctggtgaggatgagacccgtcccgagaagggtgactttcctcttgggagattcctatcacttttagagacccggacttccccgttctattcagctcctggaaagaaactggggaggctctttcaaaaggctcaggcttgtcaaatgagttgggcctgctcagggagttggtgtgctggatgacagagattccagttccgtgtctctgcagttctatcttgtcctgggctgctgaacttatctgttgttccatgatggtcgacagcttgggatccatggtctgctcagggcccctggcaacaaggtgaatatgggagttttgcaactgtatatttttatgctgctggtcacttcttatggtaacattatgtttaggcaaactgggattacagcccagagcattctgaaactgaaggccttcagaactttttggagatgttccactttcattttgctgaagttcttcatcatccccaacacttttcattttcctcctttttcttatctggggcgtctgttcccagatgccggaggacccagcgactctgtagtgtagaatctgaggctgcagaccgccgggcacagggctgtgctcaggttctctcatggctacctttgtttttggtccatgtaactcagaacagtaaaatttcttatgattttcaaaattttccagtttcctatacctgtttctacaagtttcacactcaaacattgtccctcgcccttgatgagacttctttttttctatatgtgggccttgtgccagtgccttgctcctcactgacatggcttcaccagcagcatggcatccttggtggctctcatccagggactgtccagtaccaagaacatgactttcatttgctgaagagtcttctatggctgcttgtctcacaagtgtacggggatgcccactctggggcacaggagcgttaggtcccgatacaaagacatcatcatagaaagcgccaattttgtcatcaaatgactgacttcctcttagtggatgaggaggaggtattatatttgcaggtactgctgaataacctgtggtcggcatggaattacttcttgtgataggtaaacagtcaagtgaaggtacagacagaagaaacacttgctttgatttttcagtaggggtgaaaggtgacttcggtatatcagagcttgaacttgttctccgtcccactggttttaaatcaaactggaaagaatctttaaatatgtatgatttgggggaatcaatgcttcctcgtcttgacagtgaggttctccgcggcttcacactatccagttgcttgtcatctaccaaagcttcattgtctgagataagcttcgatatccgctcctcaagtgtttttgtggccaaaggtgggcgcatctgacctggtaaaagcaatgccttttcccctgtgggcaaagcagagggtgttgacgtggtgacaagagctgcagagggtccgttactccttccagagtcttgttctgtgctgggtaaccttctggcaaagggagttggtggactcactgtttgatcggcactttcagaacgtgaaaagtaaccagaatccgtacttcctaaacttcgaggactcaggagctttccttgctgctcttgggagtaatcggtagcctgctgcctttgtagctgggcgtgtaccgttcctacgtgagagtcttgctttccttccagtggattcatgtcgcctttctggtgggaattctcattagtctccaacctggagactccaccctgggacatgttggctgaaagtggctgtacgtttgtcacctgaaggtccttctgcttttgtgcactagaaagttcaggcttgggatccatggcctttggactgtcagttcttaagggggacacagtgacatggtggaccacaactttcggtaactctgtcacagcttgtgattctgcagatctgtcctgtagcaaaaagtcacctatcacattttctggactgcttggagtgaagcttgattttagtaaagtttcagcatttgacatcctctttattatgtgcacaggctgcagctccatggcgcccaggtcatgctgtctctcatcagtggcgccttcctcctcgctctccccactgtcttctacgtctgaatgaatactaagtgctttgggggactcgtgggacaagaacaagccaccagcatctggttgcaagacaagacccagtttgatagtatgtgcgtgggatttcttgtgcttatacagattacttttagtcttaaatgaaaatccacaagtcacacagggatagggtcgctctccagtgtgggagcggatatgctttaaaagcacactaggctttgcacatgctctattgcaatactcacaaatatattttccttgtttttttggcttctgatctttcagaagaagattgcacatttgctctacgctttgattaacaacagaggcaacatgagttgaattatagattggcatggggggcgactgtgtagaattagccggacttattgacaaaggtgaagcagaatccatttgctggttttgaggagtaacctgagatctactggaaggtgaagttaggcctacagatgatgtcactgctatattataaacctgttcaagtttggcattctcttgattttgcagatttgtcagtgatcctgtgaaacctgaacaccccggaagctgttgattatgttggttggatttgggaacaaagtgttcatgttgatgatacaaatgagaagctgactgcattgccccttgctcattcttctgagcagcagacatatggactgtgtatgaggtacaagaagactgtgattcagcaaccaattcctgtgaagtctgatttggggcatccattgaactgttttttaatttgggaggggaacgtgcagttttatttggcctcagtttttctgtcttaattgcacaaggtgagcccttttgtgacaaggtgctcagttctggctccattgctttcagtaagacatcgaatgcagtgtttgtataggagggggacgtagtgccacaatgagaagagatgcattcgctattgtcagtcctggttttacttgacaaggaacttgagtcacattgttcatcgaggtcactgaatttggcaggatcagcgccttcggatctccatctacgcagttcagatggttgctgcagaaacaagggcttctttggggagacagattcttcagattttgaggcttcagcaattattccaggtgtttctccattttgtttggtaaactgcttcccattttttacaggaatataattctgtttcttgtgagactccgaagcactatgaagaacggcgaaagatgactcttctgtattttgtttatgttttgcctgaagaggatttctcagtggggattttggtatttttttcaggtgattctcagctacgatctttttgcgtttcacacctttaagggattccgaagttcctttaacaccagcctgtaagatttctttttttgaaacttctgccccattaagttctttttgtgcttcttcaattttgtcaagaccatgcggaagagccaccccgtgcagtccagtgacccttctccacggaacccaggacaacatgctaagcctttcttctgaacaccaagtgctgctctcatgctcttccaaaattcttcaacctcacaaaggataggtcggtgtcaaaacggcacccaccacgtttcctcttagatttctgggatgaatttgtttagttcgaggcatcttctttgactcagggccttctttttcttcttaaaaactgcagataaagcaagccaccaaaaggcagctccataaactcaacatacatcaattaatccatgtgctgctgccaggacgcccggcggagccgctgccgctgcagccggccctggagctgcgctgctgatggcggcggccgcggctcgggatctccgcgacccccgcgcggcggcggcggcggcgcctgggatccctccttcacttgacaaccccaaacacaaacataacctcctccggcggccgccgctccccggtcccccgctccgtccgccaccctgccgccgcccagcagccgc

SEQ ID NO: 9720 - RNA, 5805 nt, Homo sapiens
  source 1..5805: mol_type = other RNA
atgcacctgggcaaggattctgatagagaagaattttggctcatctctgaaaaaacattttcacatagaaattccttctctgggtttggcaaagcattctgatgacctttttgtaatgttggcacagaattttgttcttcactgattggcactacactatgattagtctggcaaattggctgattgggcagatcttgggtcactagtatttgtggcagggatgtgagtgtagcaaaacagtaagcaggaacactactctgcaggcgtatgggcagcatgaatgatgatggcaccttctgcacctgacttccaaggggcctgagctctggtggtagcagaggatgcgaattagacatgctgtcaattaatttggttggtaatgttgctgatgtcacacaatgatctgttccaactggatctgaaataacttgatttggcaaagaatgcacaggattagaagagcaagatgggcctgaagtgaaaacctgacaatgcaattggtatttgggagcaaagcaatcctcacttttagaagacccagataaaacagaatttttatctggcttgctaccctgcgtagacacttgcagagatagctgtgtgctctggtggctaggcggtgcatggatttgatttaacaaattgatatcacagagctgttgaacaggaaaaacgttggtagagctggagtttgatgtttctgcctgcagatccttaacctgagtctgagagtgcaaagtatttgcagaaaactcagctaaagatgtactagtgagctgaggcccctgatatggcactgcattcacactgggaagagcagtattttggaaagatgttgggtgtacaggagacagatgactatctggggctatgtttaaagatatttgccgtaccagtgggcctctccttctttctaagagaggcacatgcccagtcactcccactcgagaaggtgaagatggaggctgcaattcagtaagtggtgttgtctggggtggggtgatgcttccacaatcgaatgatttgcttctgagatcagagacctccattgacgtttgcgtgcaattaatctgttctgatgcagtacgcctcatttcccggtgacatccaggaacattcagagtattcaagccagctggaatcataagaaactcggctttatttagaaaatcgattttgggggaagcctccgttttagaaacgtcctctatgtctaaagaggctgagaaacttgaagtgtgagataaactgctctccctacttagactcctggagagagtggaatcaaagctcgattctgttgaggaatgttctatctcagccagacggagccttttctttttgggtggcagtttctctgttggcaattttgacaaggtttcactacgctggggccaactgaacttctctgacttttcttgatcatggcattgagcttccaggtctcgatctggttcttctgtgaccaaaatctctggaacttggatgttgtgctgccggacaagtcttgagggctgtcctaacacatgtcgttcacttggactctttctggagctttcctgaagttctcctctgagagcgtctgatagtgcaagctggtgaggatgagacccgtcccgagaagggtgactttcctcttgggagattcctatcacttttagagacccggacttccccgttctattcagctcctggaaagaaactggggaggctctttcaaaaggctcaggcttgtcaaatgagttgggcctgctcagggagttggtgtgctggatgacagagattccagttccgtgtctctgcagttctatcttgtcctgggctgctgaacttatctgttgttccatgatggtcgacagcttgggatccatggtctgctcagggcccctggcaacaaggtgaatatgggagttttgcaactgtatatttttatgctgctggtcacttcttatggtaacattatgtttaggcaaactgggattacagcccagagcattctgaaactgaaggccttcagaactttttggagatgttccactttcattttgctgaagttcttcatcatccccaacacttttcattttcctcctttttcttatctggggcgtctgttcccagatgccggaggacccagcgactctgtagtgtagaatctgaggctgcagaccgccgggcacagggctgtgctcaggttctctcatggctacctttgtttttggtccatgtaactcagaacagtaaaatttcttatgattttcaaaattttccagtttcctatacctgtttctacaagtttcacactcaaacattgtccctcgcccttgatgagacttctttttttctatatgtgggccttgtgccagtgccttgctcctcactgacatggcttcaccagcagcatggcatccttggtggctctcatccagggactgtccagtaccaagaacatgactttcatttgctgaagagtcttctatggctgcttgtctcacaagtgtacggggatgcccactctggggcacaggagcgttaggtcccgatacaaagacatcatcatagaaagcgccaattttgtcatcaaatgactgacttcctcttagtggatgaggaggaggtattatatttgcaggtactgctgaataacctgtggtcggcatggaattacttcttgtgataggtaaacagtcaagtgaaggtacagacagaagaaacacttgctttgatttttcagtaggggtgaaaggtgacttcggtatatcagagcttgaacttgttctccgtcccactggttttaaatcaaactggaaagaatctttaaatatgtatgatttgggggaatcaatgcttcctcgtcttgacagtgaggttctccgcggcttcacactatccagttgcttgtcatctaccaaagcttcattgtctgagataagcttcgatatccgctcctcaagtgtttttgtggccaaaggtgggcgcatctgacctggtaaaagcaatgccttttcccctgtgggcaaagcagagggtgttgacgtggtgacaagagctgcagagggtccgttactccttccagagtcttgttctgtgctgggtaaccttctggcaaagggagttggtggactcactgtttgatcggcactttcagaacgtgaaaagtaaccagaatccgtacttcctaaacttcgaggactcaggagctttccttgctgctcttgggagtaatcggtagcctgctgcctttgtagctgggcgtgtaccgttcctacgtgagagtcttgctttccttccagtggattcatgtcgcctttctggtgggaattctcattagtctccaacctggagactccaccctgggacatgttggctgaaagtggctgtacgtttgtcacctgaaggtccttctgcttttgtgcactagaaagttcaggcttgggatccatggcctttggactgtcagttcttaagggggacacagtgacatggtggaccacaactttcggtaactctgtcacagcttgtgattctgcagatctgtcctgtagcaaaaagtcacctatcacattttctggactgcttggagtgaagcttgattttagtaaagtttcagcatttgacatcctctttattatgtgcacaggctgcagctccatggcgcccaggtcatgctgtctctcatcagtggcgccttcctcctcgctctccccactgtcttctacgtctgaatgaatactaagtgctttgggggactcgtgggacaagaacaagccaccagcatctggttgcaagacaagacccagtttgatagtatgtgcgtgggatttcttgtgcttatacagattacttttagtcttaaatgaaaatccacaagtcacacagggatagggtcgctctccagtgtgggagcggatatgctttaaaagcacactaggctttgcacatgctctattgcaatactcacaaatatattttccttgtttttttggcttctgatctttcagaagaagattgcacatttgctctacgctttgattaacaacagaggcaacatgagttgaattatagattggcatggggggcgactgtgtagaattagccggacttattgacaaaggtgaagcagaatccatttgctggttttgaggagtaacctgagatctactggaaggtgaagttaggcctacagatgatgtcactgctatattataaacctgttcaagtttggcattctcttgattttgcagatttgtcagtgatcctgtgaaacctgaacaccccggaagctgttgattatgttggttggatttgggaacaaagtgttcatgttgatgatacaaatgagaagctgactgcattgccccttgctcattcttctgagcagcagacatatggactgtgtatgaggtacaagaagactgtgattcagcaaccaattcctgtgaagtctgatttggggcatccattgaactgttttttaatttgggaggggaacgtgcagttttatttggcctcagtttttctgtcttaattgcacaaggtgagcccttttgtgacaaggtgctcagttctggctccattgctttcagtaagacatcgaatgcagtgtttgtataggagggggacgtagtgccacaatgagaagagatgcattcgctattgtcagtcctggttttacttgacaaggaacttgagtcacattgttcatcgaggtcactgaatttggcaggatcagcgccttcggatctccatctacgcagttcagatggttgctgcagaaacaagggcttctttggggagacagattcttcagattttgaggcttcagcaattattccaggtgtttctccattttgtttggtaaactgcttcccattttttacaggaatataattctgtttcttgtgagactccgaagcactatgaagaacggcgaaagatgactcttctgtattttgtttatgttttgcctgaagaggatttctcagtggggattttggtatttttttcaggtgattctcagctacgatctttttgcgtttcacacctttaagggattccgaagttcctttaacaccagcctgtaagatttctttttttgaaacttctgccccattaagttctttttgtgcttcttcaattttgtcaagaccatgcggaagagccaccccgtgcagtccagtgacccttctccacggaacccaggacaacatgctaagcctttcttctgaacaccaagtgctgctctcatgctcttccaaaattcttcaacctcacaaaggataggtcggtgtcaaaacggcacccaccacgtttcctcttagatttctgggatgaatttgtttagttcgaggcatcttctttgactcagggccttctttttcttcttaaaaactgcagataaagcaagccaccaaaaggcagctccataaactcaacatacatcaattaatccatgtgctgtgcctccactttacaccaacagaagcttgtgttcaggccttgccctctggaagattacaaattaatggagacaggataaacacatggaaaaatacctagagggaaaaaaagatataagaggcttataaacagagccaattaaagttatacagttatttacatgatcgctgagaggcttctgcttgagtagaggacggggtgagcagagtcccatcctgggggtgagttctcagtgggatattgaaggagagaaagttcacgatttggcagtggtggaagtacagcattctagaggagggaaataacttgaaggtgagagcaagtgaactgtgtgtgatggtttttcca

SEQ ID NO: 9721 - RNA, 6961 nt, Homo sapiens
  source 1..6961: mol_type = other RNA
atgcacctgggcaaggattctgatagagaagaattttggctcatctctgaaaaaacattttcacatagaaattccttctctgggtttggcaaagcattctgatgacctttttgtaatgttggcacagaattttgttcttcactgattggcactacactatgattagtctggcaaattggctgattgggcagatcttgggtcactagtatttgtggcagggatgtgagtgtagcaaaacagtaagcaggaacactactctgcaggcgtatgggcagcatgaatgatgatggcaccttctgcacctgacttccaaggggcctgagctctggtggtagcagaggatgcgaattagacatgctgtcaattaatttggttggtaatgttgctgatgtcacacaatgatctgttccaactggatctgaaataacttgatttggcaaagaatgcacaggattagaagagcaagatgggcctgaagtgaaaacctgacaatgcaattggtatttgggagcaaagcaatcctcacttttagaagacccagataaaacagaatttttatctggcttgctaccctgcgtagacacttgcagagatagctgtgtgctctggtggctaggcggtgcatggatttgatttaacaaattgatatcacagagctgttgaacaggaaaaacgttggtagagctggagtttgatgtttctgcctgcagatccttaacctgagtctgagagtgcaaagtatttgcagaaaactcagctaaagatgtactagtgagctgaggcccctgatatggcactgcattcacactgggaagagcagtattttggaaagatgttgggtgtacaggagacagatgactatctggggctatgtttaaagatatttgccgtaccagtgggcctctccttctttctaagagaggcacatgcccagtcactcccactcgagaaggtgaagatggaggctgcaattcagtaagtggtgttgtctggggtggggtgatgcttccacaatcgaatgatttgcttctgagatcagagacctccattgacgtttgcgtgcaattaatctgttctgatgcagtacgcctcatttcccggtgacatccaggaacattcagagtattcaagccagctggaatcataagaaactcggctttatttagaaaatcgattttgggggaagcctccgttttagaaacgtcctctatgtctaaagaggctgagaaacttgaagtgtgagataaactgctctccctacttagactcctggagagagtggaatcaaagctcgattctgttgaggaatgttctatctcagccagacggagccttttctttttgggtggcagtttctctgttggcaattttgacaaggtttcactacgctggggccaactgaacttctctgacttttcttgatcatggcattgagcttccaggtctcgatctggttcttctgtgaccaaaatctctggaacttggatgttgtgctgccggacaagtcttgagggctgtcctaacacatgtcgttcacttggactctttctggagctttcctgaagttctcctctgagagcgtctgatagtgcaagctggtgaggatgagacccgtcccgagaagggtgactttcctcttgggagattcctatcacttttagagacccggacttccccgttctattcagctcctggaaagaaactggggaggctctttcaaaaggctcaggcttgtcaaatgagttgggcctgctcagggagttggtgtgctggatgacagagattccagttccgtgtctctgcagttctatcttgtcctgggctgctgaacttatctgttgttccatgatggtcgacagcttgggatccatggtctgctcagggcccctggcaacaaggtgaatatgggagttttgcaactgtatatttttatgctgctggtcacttcttatggtaacattatgtttaggcaaactgggattacagcccagagcattctgaaactgaaggccttcagaactttttggagatgttccactttcattttgctgaagttcttcatcatccccaacacttttcattttcctcctttttcttatctggggcgtctgttcccagatgccggaggacccagcgactctgtagtgtagaatctgaggctgcagaccgccgggcacagggctgtgctcaggttctctcatggctacctttgtttttggtccatgtaactcagaacagtaaaatttcttatgattttcaaaattttccagtttcctatacctgtttctacaagtttcacactcaaacattgtccctcgcccttgatgagacttctttttttctatatgtgggccttgtgccagtgccttgctcctcactgacatggcttcaccagcagcatggcatccttggtggctctcatccagggactgtccagtaccaagaacatgactttcatttgctgaagagtcttctatggctgcttgtctcacaagtgtacggggatgcccactctggggcacaggagcgttaggtcccgatacaaagacatcatcatagaaagcgccaattttgtcatcaaatgactgacttcctcttagtggatgaggaggaggtattatatttgcaggtactgctgaataacctgtggtcggcatggaattacttcttgtgataggtaaacagtcaagtgaaggtacagacagaagaaacacttgctttgatttttcagtaggggtgaaaggtgacttcggtatatcagagcttgaacttgttctccgtcccactggttttaaatcaaactggaaagaatctttaaatatgtatgatttgggggaatcaatgcttcctcgtcttgacagtgaggttctccgcggcttcacactatccagttgcttgtcatctaccaaagcttcattgtctgagataagcttcgatatccgctcctcaagtgtttttgtggccaaaggtgggcgcatctgacctggtaaaagcaatgccttttcccctgtgggcaaagcagagggtgttgacgtggtgacaagagctgcagagggtccgttactccttccagagtcttgttctgtgctgggtaaccttctggcaaagggagttggtggactcactgtttgatcggcactttcagaacgtgaaaagtaaccagaatccgtacttcctaaacttcgaggactcaggagctttccttgctgctcttgggagtaatcggtagcctgctgcctttgtagctgggcgtgtaccgttcctacgtgagagtcttgctttccttccagtggattcatgtcgcctttctggtgggaattctcattagtctccaacctggagactccaccctgggacatgttggctgaaagtggctgtacgtttgtcacctgaaggtccttctgcttttgtgcactagaaagttcaggcttgggatccatggcctttggactgtcagttcttaagggggacacagtgacatggtggaccacaactttcggtaactctgtcacagcttgtgattctgcagatctgtcctgtagcaaaaagtcacctatcacattttctggactgcttggagtgaagcttgattttagtaaagtttcagcatttgacatcctctttattatgtgcacaggctgcagctccatggcgcccaggtcatgctgtctctcatcagtggcgccttcctcctcgctctccccactgtcttctacgtctgaatgaatactaagtgctttgggggactcgtgggacaagaacaagccaccagcatctggttgcaagacaagacccagtttgatagtatgtgcgtgggatttcttgtgcttatacagattacttttagtcttaaatgaaaatccacaagtcacacagggatagggtcgctctccagtgtgggagcggatatgctttaaaagcacactaggctttgcacatgctctattgcaatactcacaaatatattttccttgtttttttggcttctgatctttcagaagaagattgcacatttgctctacgctttgattaacaacagaggcaacatgagttgaattatagattggcatggggggcgactgtgtagaattagccggacttattgacaaaggtgaagcagaatccatttgctggttttgaggagtaacctgagatctactggaaggtgaagttaggcctacagatgatgtcactgctatattataaacctgttcaagtttggcattctcttgattttgcagatttgtcagtgatcctgtgaaacctgaacaccccggaagctgttgattatgttggttggatttgggaacaaagtgttcatgttgatgatacaaatgagaagctgactgcattgccccttgctcattcttctgagcagcagacatatggactgtgtatgaggtacaagaagactgtgattcagcaaccaattcctgtgaagtctgatttggggcatccattgaactgttttttaatttgggaggggaacgtgcagttttatttggcctcagtttttctgtcttaattgcacaaggtgagcccttttgtgacaaggtgctcagttctggctccattgctttcagtaagacatcgaatgcagtgtttgtataggagggggacgtagtgccacaatgagaagagatgcattcgctattgtcagtcctggttttacttgacaaggaacttgagtcacattgttcatcgaggtcactgaatttggcaggatcagcgccttcggatctccatctacgcagttcagatggttgctgcagaaacaagggcttctttggggagacagattcttcagattttgaggcttcagcaattattccaggtgtttctccattttgtttggtaaactgcttcccattttttacaggaatataattctgtttcttgtgagactccgaagcactatgaagaacggcgaaagatgactcttctgtattttgtttatgttttgcctgaagaggatttctcagtggggattttggtatttttttcaggtgattctcagctacgatctttttgcgtttcacacctttaagggattccgaagttcctttaacaccagcctgtaagatttctttttttgaaacttctgccccattaagttctttttgtgcttcttcaattttgtcagccatgacaggtcggccatccccattatctgtgccgccgcggcacacctgagctccctgccccttcacgtcacatctaggagcagctctaaggcagactctcgctcatgggctgcctcctggaagtcctcccccactacctctccatggcaaccgcagccacagagaagccagtccatctcttacgcaaatgaaaggaggccacaaatgtcagcagtcacaacatccccattttccctccctacttaatttccttcttaaagtcacagtaatgcattcttcttattctgcatccgagagtaccttcccaaccgtttaatggccaggaaagcaacttaggaaaatcagagttaaaaatccatctgtgtgaccacttacataacatgactgagaatccaaagatgattatgatttgctgagtttcatttactgacacagtatctcagcaagccccctttatgtctcagcatcctagtatttgagataagagtcctttaagatattaactatcctgtaatttggctttcttaaaaacgacagagagagagaggccatccattatgacagtcaagaaacaatcagtacttaatatgcattgtttcttttgcagattctcatttatttagaaaagtcaaggttttaaaaaatatttttacttttaaaccaaatcatcaactatctaattctacaggagggaaaaactgaacagattatcattcattattcaattgttatcaggtttagtttatactgtaattgtctgaagttttatttcccagatatatatttaaagaagcaaatataatggctagttacacttcatatggctacagagattggaaagcagatgtaaatccccattaacaaaatcatgcttacaataactgtttaatatatagatgtcagattttaaagtatgttttaatccatgggatgcaccaaagtatcaaattctgtaagtggttataaacatgtgatggtctaataaaaagaattccaattgaaatagcttggaacaagatactactggtgaacaatataaacgtggtgggtttaatattctccaaaacatgtattcgaaatcaattgaaatccaaaacagttatgtttacatgaaaaacaatacaagagaattagaacattaaaaagtacatatatatgtatacatgtatatgcatacacattttttagttgtccaatgaaaagggcaatttaaaaacttgaattcttcagcaaaacatttactaagtatctaccaatgtgctacgtaccctacagtttagggacacagagacatgaggcattttcatggagggccactcagaggcagtgggagctgtacctcaagcagccccaacccatcccagctgagtattccaggaggctgcccagagggactagaggtgaatctcaggatcaagtttcagtccacagcagaaaaagactcaagagattcagggaaaagcatgatggttagaaacagcacagtaggcgaggagaaccccaggtaggtggcaatgcagggagcaccaccggagggatgtggcagaagaagcagtcaagatcatggacacagtaacgtgaaaggaatctaagcctttatcttgaggtttagggttagagtatagtgttctagataacacaataacacaatcacattacaaattactcaaattattcattgctgttggttctaaatgtttagcgggaatccccacccaacctctgtaccccgccccccaaaaaatgtaggataagaaagtatgaatgttggctgggcgcagtggctcacgcctgtaattccagcactttgggaggcc

SEQ ID NO: 9722 - RNA, 6230 nt, Homo sapiens
  source 1..6230: mol_type = other RNA
atgcacctgggcaaggattctgatagagaagaattttggctcatctctgaaaaaacattttcacatagaaattccttctctgggtttggcaaagcattctgatgacctttttgtaatgttggcacagaattttgttcttcactgattggcactacactatgattagtctggcaaattggctgattgggcagatcttgggtcactagtatttgtggcagggatgtgagtgtagcaaaacagtaagcaggaacactactctgcaggcgtatgggcagcatgaatgatgatggcaccttctgcacctgacttccaaggggcctgagctctggtggtagcagaggatgcgaattagacatgctgtcaattaatttggttggtaatgttgctgatgtcacacaatgatctgttccaactggatctgaaataacttgatttggcaaagaatgcacaggattagaagagcaagatgggcctgaagtgaaaacctgacaatgcaattggtatttgggagcaaagcaatcctcacttttagaagacccagataaaacagaatttttatctggcttgctaccctgcgtagacacttgcagagatagctgtgtgctctggtggctaggcggtgcatggatttgatttaacaaattgatatcacagagctgttgaacaggaaaaacgttggtagagctggagtttgatgtttctgcctgcagatccttaacctgagtctgagagtgcaaagtatttgcagaaaactcagctaaagatgtactagtgagctgaggcccctgatatggcactgcattcacactgggaagagcagtattttggaaagatgttgggtgtacaggagacagatgactatctggggctatgtttaaagatatttgccgtaccagtgggcctctccttctttctaagagaggcacatgcccagtcactcccactcgagaaggtgaagatggaggctgcaattcagtaagtggtgttgtctggggtggggtgatgcttccacaatcgaatgatttgcttctgagatcagagacctccattgacgtttgcgtgcaattaatctgttctgatgcagtacgcctcatttcccggtgacatccaggaacattcagagtattcaagccagctggaatcataagaaactcggctttatttagaaaatcgattttgggggaagcctccgttttagaaacgtcctctatgtctaaagaggctgagaaacttgaagtgtgagataaactgctctccctacttagactcctggagagagtggaatcaaagctcgattctgttgaggaatgttctatctcagccagacggagccttttctttttgggtggcagtttctctgttggcaattttgacaaggtttcactacgctggggccaactgaacttctctgacttttcttgatcatggcattgagcttccaggtctcgatctggttcttctgtgaccaaaatctctggaacttggatgttgtgctgccggacaagtcttgagggctgtcctaacacatgtcgttcacttggactctttctggagctttcctgaagttctcctctgagagcgtctgatagtgcaagctggtgaggatgagacccgtcccgagaagggtgactttcctcttgggagattcctatcacttttagagacccggacttccccgttctattcagctcctggaaagaaactggggaggctctttcaaaaggctcaggcttgtcaaatgagttgggcctgctcagggagttggtgtgctggatgacagagattccagttccgtgtctctgcagttctatcttgtcctgggctgctgaacttatctgttgttccatgatggtcgacagcttgggatccatggtctgctcagggcccctggcaacaaggtgaatatgggagttttgcaactgtatatttttatgctgctggtcacttcttatggtaacattatgtttaggcaaactgggattacagcccagagcattctgaaactgaaggccttcagaactttttggagatgttccactttcattttgctgaagttcttcatcatccccaacacttttcattttcctcctttttcttatctggggcgtctgttcccagatgccggaggacccagcgactctgtagtgtagaatctgaggctgcagaccgccgggcacagggctgtgctcaggttctctcatggctacctttgtttttggtccatgtaactcagaacagtaaaatttcttatgattttcaaaattttccagtttcctatacctgtttctacaagtttcacactcaaacattgtccctcgcccttgatgagacttctttttttctatatgtgggccttgtgccagtgccttgctcctcactgacatggcttcaccagcagcatggcatccttggtggctctcatccagggactgtccagtaccaagaacatgactttcatttgctgaagagtcttctatggctgcttgtctcacaagtgtacggggatgcccactctggggcacaggagcgttaggtcccgatacaaagacatcatcatagaaagcgccaattttgtcatcaaatgactgacttcctcttagtggatgaggaggaggtattatatttgcaggtactgctgaataacctgtggtcggcatggaattacttcttgtgataggtaaacagtcaagtgaaggtacagacagaagaaacacttgctttgatttttcagtaggggtgaaaggtgacttcggtatatcagagcttgaacttgttctccgtcccactggttttaaatcaaactggaaagaatctttaaatatgtatgatttgggggaatcaatgcttcctcgtcttgacagtgaggttctccgcggcttcacactatccagttgcttgtcatctaccaaagcttcattgtctgagataagcttcgatatccgctcctcaagtgtttttgtggccaaaggtgggcgcatctgacctggtaaaagcaatgccttttcccctgtgggcaaagcagagggtgttgacgtggtgacaagagctgcagagggtccgttactccttccagagtcttgttctgtgctgggtaaccttctggcaaagggagttggtggactcactgtttgatcggcactttcagaacgtgaaaagtaaccagaatccgtacttcctaaacttcgaggactcaggagctttccttgctgctcttgggagtaatcggtagcctgctgcctttgtagctgggcgtgtaccgttcctacgtgagagtcttgctttccttccagtggattcatgtcgcctttctggtgggaattctcattagtctccaacctggagactccaccctgggacatgttggctgaaagtggctgtacgtttgtcacctgaaggtccttctgcttttgtgcactagaaagttcaggcttgggatccatggcctttggactgtcagttcttaagggggacacagtgacatggtggaccacaactttcggtaactctgtcacagcttgtgattctgcagatctgtcctgtagcaaaaagtcacctatcacattttctggactgcttggagtgaagcttgattttagtaaagtttcagcatttgacatcctctttattatgtgcacaggctgcagctccatggcgcccaggtcatgctgtctctcatcagtggcgccttcctcctcgctctccccactgtcttctacgtctgaatgaatactaagtgctttgggggactcgtgggacaagaacaagccaccagcatctggttgcaagacaagacccagtttgatagtatgtgcgtgggatttcttgtgcttatacagattacttttagtcttaaatgaaaatccacaagtcacacagggatagggtcgctctccagtgtgggagcggatatgctttaaaagcacactaggctttgcacatgctctattgcaatactcacaaatatattttccttgtttttttggcttctgatctttcagaagaagattgcacatttgctctacgctttgattaacaacagaggcaacatgagttgaattatagattggcatggggggcgactgtgtagaattagccggacttattgacaaaggtgaagcagaatccatttgctggttttgaggagtaacctgagatctactggaaggtgaagttaggcctacagatgatgtcactgctatattataaacctgttcaagtttggcattctcttgattttgcagatttgtcagtgatcctgtgaaacctgaacaccccggaagctgttgattatgttggttggatttgggaacaaagtgttcatgttgatgatacaaatgagaagctgactgcattgccccttgctcattcttctgagcagcagacatatggactgtgtatgaggtacaagaagactgtgattcagcaaccaattcctgtgaagtctgatttggggcatccattgaactgttttttaatttgggaggggaacgtgcagttttatttggcctcagtttttctgtcttaattgcacaaggtgagcccttttgtgacaaggtgctcagttctggctccattgctttcagtaagacatcgaatgcagtgtttgtataggagggggacgtagtgccacaatgagaagagatgcattcgctattgtcagtcctggttttacttgacaaggaacttgagtcacattgttcatcgaggtcactgaatttggcaggatcagcgccttcggatctccatctacgcagttcagatggttgctgcagaaacaagggcttctttggggagacagattcttcagattttgaggcttcagcaattattccaggtgtttctccattttgtttggtaaactgcttcccattttttacaggaatataattctgtttcttgtgagactccgaagcactatgaagaacggcgaaagatgactcttctgtattttgtttatgttttgcctgaagaggatttctcagtggggattttggtatttttttcaggtgattctcagctacgatctttttgcgtttcacacctttaagggattccgaagttcctttaacaccagcctgtaagatttctttttttgaaacttctgccccattaagttctttttgtgcttcttcaattttgtctcttagatttctgggatgaatttgtttagttcgaggcatcttctttgactcagggccttctttttcttcttaaaaactgcagataaagcaagccaccaaaaggcagctccataaactcaacatacatcaattaatccatgtgccgaactgcaacacaaaagtctgatccaaagcttcctgggtttaacttttaattttaaaaacaaaaaagcagaaaccaaaagcctcctaggttggaagtgggcgtgagaggaaatgctagagggaggcgcttcattccccgggctgcctgtgcccccctttctggcccctgcccggggctttgatgttatctagtgcaccgcctccatcggtttctaccttgggctctgcgccgccgagaagatagacagatcttccgcacttcacttgcaggttctgagagaggcaagcaggtagtcgcgggaaaggacccacactccttagccccgcagtgagagaggaacatttgcacgggcttcctgttgctacctggactgaaatgaacaatccacccctctagtgatcctggagacttgcaccgtatggtctttcctgctagacgcacagcgggaggcctcctacattagattcattttccctccacccgtagcacaaacttgtaagatggtggtggagtatgtttcctgaggctttgttcgggttttagatctcagtttggaaggtaaatattatttcccttctgagacagtcctgcagcctgtgcctccactttacaccaacagaagcttgtgttcaggccttgccctctggaagattacaaattaatggagacaggataaacacatggaaaaatacctagagggaaaaaaagatataagaggcttataaacagagccaattaaagttatacagttatttacatgatcgctgagaggcttctgcttgagtagaggacggggtgagcagagtcccatcctgggggtgagttctcagtgggatattgaaggagagaaagttcacgatttggcagtggtggaagtacagcattctagaggagggaaataacttgaaggtgagagcaagtgaactgtgtgtgatggtttttcc

SEQ ID NO: 9723 - RNA, 5390 nt, Homo sapiens
  source 1..5390: mol_type = other RNA
atgcacctgggcaaggattctgatagagaagaattttggctcatctctgaaaaaacattttcacatagaaattccttctctgggtttggcaaagcattctgatgacctttttgtaatgttggcacagaattttgttcttcactgattggcactacactatgattagtctggcaaattggctgattgggcagatcttgggtcactagtatttgtggcagggatgtgagtgtagcaaaacagtaagcaggaacactactctgcaggcgtatgggcagcatgaatgatgatggcaccttctgcacctgacttccaaggggcctgagctctggtggtagcagaggatgcgaattagacatgctgtcaattaatttggttggtaatgttgctgatgtcacacaatgatctgttccaactggatctgaaataacttgatttggcaaagaatgcacaggattagaagagcaagatgggcctgaagtgaaaacctgacaatgcaattggtatttgggagcaaagcaatcctcacttttagaagacccagataaaacagaatttttatctggcttgctaccctgcgtagacacttgcagagatagctgtgtgctctggtggctaggcggtgcatggatttgatttaacaaattgatatcacagagctgttgaacaggaaaaacgttggtagagctggagtttgatgtttctgcctgcagatccttaacctgagtctgagagtgcaaagtatttgcagaaaactcagctaaagatgtactagtgagctgaggcccctgatatggcactgcattcacactgggaagagcagtattttggaaagatgttgggtgtacaggagacagatgactatctggggctatgtttaaagatatttgccgtaccagtgggcctctccttctttctaagagaggcacatgcccagtcactcccactcgagaaggtgaagatggaggctgcaattcagtaagtggtgttgtctggggtggggtgatgcttccacaatcgaatgatttgcttctgagatcagagacctccattgacgtttgcgtgcaattaatctgttctgatgcagtacgcctcatttcccggtgacatccaggaacattcagagtattcaagccagctggaatcataagaaactcggctttatttagaaaatcgattttgggggaagcctccgttttagaaacgtcctctatgtctaaagaggctgagaaacttgaagtgtgagataaactgctctccctacttagactcctggagagagtggaatcaaagctcgattctgttgaggaatgttctatctcagccagacggagccttttctttttgggtggcagtttctctgttggcaattttgacaaggtttcactacgctggggccaactgaacttctctgacttttcttgatcatggcattgagcttccaggtctcgatctggttcttctgtgaccaaaatctctggaacttggatgttgtgctgccggacaagtcttgagggctgtcctaacacatgtcgttcacttggactctttctggagctttcctgaagttctcctctgagagcgtctgatagtgcaagctggtgaggatgagacccgtcccgagaagggtgactttcctcttgggagattcctatcacttttagagacccggacttccccgttctattcagctcctggaaagaaactggggaggctctttcaaaaggctcaggcttgtcaaatgagttgggcctgctcagggagttggtgtgctggatgacagagattccagttccgtgtctctgcagttctatcttgtcctgggctgctgaacttatctgttgttccatgatggtcgacagcttgggatccatggtctgctcagggcccctggcaacaaggtgaatatgggagttttgcaactgtatatttttatgctgctggtcacttcttatggtaacattatgtttaggcaaactgggattacagcccagagcattctgaaactgaaggccttcagaactttttggagatgttccactttcattttgctgaagttcttcatcatccccaacacttttcattttcctcctttttcttatctggggcgtctgttcccagatgccggaggacccagcgactctgtagtgtagaatctgaggctgcagaccgccgggcacagggctgtgctcaggttctctcatggctacctttgtttttggtccatgtaactcagaacagtaaaatttcttatgattttcaaaattttccagtttcctatacctgtttctacaagtttcacactcaaacattgtccctcgcccttgatgagacttctttttttctatatgtgggccttgtgccagtgccttgctcctcactgacatggcttcaccagcagcatggcatccttggtggctctcatccagggactgtccagtaccaagaacatgactttcatttgctgaagagtcttctatggctgcttgtctcacaagtgtacggggatgcccactctggggcacaggagcgttaggtcccgatacaaagacatcatcatagaaagcgccaattttgtcatcaaatgactgacttcctcttagtggatgaggaggaggtattatatttgcaggtactgctgaataacctgtggtcggcatggaattacttcttgtgataggtaaacagtcaagtgaaggtacagacagaagaaacacttgctttgatttttcagtaggggtgaaaggtgacttcggtatatcagagcttgaacttgttctccgtcccactggttttaaatcaaactggaaagaatctttaaatatgtatgatttgggggaatcaatgcttcctcgtcttgacagtgaggttctccgcggcttcacactatccagttgcttgtcatctaccaaagcttcattgtctgagataagcttcgatatccgctcctcaagtgtttttgtggccaaaggtgggcgcatctgacctggtaaaagcaatgccttttcccctgtgggcaaagcagagggtgttgacgtggtgacaagagctgcagagggtccgttactccttccagagtcttgttctgtgctgggtaaccttctggcaaagggagttggtggactcactgtttgatcggcactttcagaacgtgaaaagtaaccagaatccgtacttcctaaacttcgaggactcaggagctttccttgctgctcttgggagtaatcggtagcctgctgcctttgtagctgggcgtgtaccgttcctacgtgagagtcttgctttccttccagtggattcatgtcgcctttctggtgggaattctcattagtctccaacctggagactccaccctgggacatgttggctgaaagtggctgtacgtttgtcacctgaaggtccttctgcttttgtgcactagaaagttcaggcttgggatccatggcctttggactgtcagttcttaagggggacacagtgacatggtggaccacaactttcggtaactctgtcacagcttgtgattctgcagatctgtcctgtagcaaaaagtcacctatcacattttctggactgcttggagtgaagcttgattttagtaaagtttcagcatttgacatcctctttattatgtgcacaggctgcagctccatggcgcccaggtcatgctgtctctcatcagtggcgccttcctcctcgctctccccactgtcttctacgtctgaatgaatactaagtgctttgggggactcgtgggacaagaacaagccaccagcatctggttgcaagacaagacccagtttgatagtatgtgcgtgggatttcttgtgcttatacagattacttttagtcttaaatgaaaatccacaagtcacacagggatagggtcgctctccagtgtgggagcggatatgctttaaaagcacactaggctttgcacatgctctattgcaatactcacaaatatattttccttgtttttttggcttctgatctttcagaagaagattgcacatttgctctacgctttgattaacaacagaggcaacatgagttgaattatagattggcatggggggcgactgtgtagaattagccggacttattgacaaaggtgaagcagaatccatttgctggttttgaggagtaacctgagatctactggaaggtgaagttaggcctacagatgatgtcactgctatattataaacctgttcaagtttggcattctcttgattttgcagatttgtcagtgatcctgtgaaacctgaacaccccggaagctgttgattatgttggttggatttgggaacaaagtgttcatgttgatgatacaaatgagaagctgactgcattgccccttgctcattcttctgagcagcagacatatggactgtgtatgaggtacaagaagactgtgattcagcaaccaattcctgtgaagtctgatttggggcatccattgaactgttttttaatttgggaggggaacgtgcagttttatttggcctcagtttttctgtcttaattgcacaaggtgagcccttttgtgacaaggtgctcagttctggctccattgctttcagtaagacatcgaatgcagtgtttgtataggagggggacgtagtgccacaatgagaagagatgcattcgctattgtcagtcctggttttacttgacaaggaacttgagtcacattgttcatcgaggtcactgaatttggcaggatcagcgccttcggatctccatctacgcagttcagatggttgctgcagaaacaagggcttctttggggagacagattcttcagattttgaggcttcagcaattattccaggtgtttctccattttgtttggtaaactgcttcccattttttacaggaatataattctgtttcttgtgagactccgaagcactatgaagaacggcgaaagatgactcttctgtattttgtttatgttttgcctgaagaggatttctcagtggggattttggtatttttttcaggtgattctcagctacgatctttttgcgtttcacacctttaagggattccgaagttcctttaacaccagcctgtaagatttctttttttgaaacttctgccccattaagttctttttgtgcttcttcaattttgtctcttagatttctgggatgaatttgtttagttcgaggcatcttctttgactcagggccttctttttcttcttaaaaactgcagataaagcaagccaccaaaaggcagctccataaactcaacatacatcaattaatccatgtgctctcccccggggcagagtagggcacgtttagcgtctttggggccggcgggaggaacgcgggccgggcggcgcgggggaggcagggcgaaggtcggaggctttcccg

SEQ ID NO: 9724 - RNA, 5371 nt, Homo sapiens
  source 1..5371: mol_type = other RNA
atgcacctgggcaaggattctgatagagaagaattttggctcatctctgaaaaaacattttcacatagaaattccttctctgggtttggcaaagcattctgatgacctttttgtaatgttggcacagaattttgttcttcactgattggcactacactatgattagtctggcaaattggctgattgggcagatcttgggtcactagtatttgtggcagggatgtgagtgtagcaaaacagtaagcaggaacactactctgcaggcgtatgggcagcatgaatgatgatggcaccttctgcacctgacttccaaggggcctgagctctggtggtagcagaggatgcgaattagacatgctgtcaattaatttggttggtaatgttgctgatgtcacacaatgatctgttccaactggatctgaaataacttgatttggcaaagaatgcacaggattagaagagcaagatgggcctgaagtgaaaacctgacaatgcaattggtatttgggagcaaagcaatcctcacttttagaagacccagataaaacagaatttttatctggcttgctaccctgcgtagacacttgcagagatagctgtgtgctctggtggctaggcggtgcatggatttgatttaacaaattgatatcacagagctgttgaacaggaaaaacgttggtagagctggagtttgatgtttctgcctgcagatccttaacctgagtctgagagtgcaaagtatttgcagaaaactcagctaaagatgtactagtgagctgaggcccctgatatggcactgcattcacactgggaagagcagtattttggaaagatgttgggtgtacaggagacagatgactatctggggctatgtttaaagatatttgccgtaccagtgggcctctccttctttctaagagaggcacatgcccagtcactcccactcgagaaggtgaagatggaggctgcaattcagtaagtggtgttgtctggggtggggtgatgcttccacaatcgaatgatttgcttctgagatcagagacctccattgacgtttgcgtgcaattaatctgttctgatgcagtacgcctcatttcccggtgacatccaggaacattcagagtattcaagccagctggaatcataagaaactcggctttatttagaaaatcgattttgggggaagcctccgttttagaaacgtcctctatgtctaaagaggctgagaaacttgaagtgtgagataaactgctctccctacttagactcctggagagagtggaatcaaagctcgattctgttgaggaatgttctatctcagccagacggagccttttctttttgggtggcagtttctctgttggcaattttgacaaggtttcactacgctggggccaactgaacttctctgacttttcttgatcatggcattgagcttccaggtctcgatctggttcttctgtgaccaaaatctctggaacttggatgttgtgctgccggacaagtcttgagggctgtcctaacacatgtcgttcacttggactctttctggagctttcctgaagttctcctctgagagcgtctgatagtgcaagctggtgaggatgagacccgtcccgagaagggtgactttcctcttgggagattcctatcacttttagagacccggacttccccgttctattcagctcctggaaagaaactggggaggctctttcaaaaggctcaggcttgtcaaatgagttgggcctgctcagggagttggtgtgctggatgacagagattccagttccgtgtctctgcagttctatcttgtcctgggctgctgaacttatctgttgttccatgatggtcgacagcttgggatccatggtctgctcagggcccctggcaacaaggtgaatatgggagttttgcaactgtatatttttatgctgctggtcacttcttatggtaacattatgtttaggcaaactgggattacagcccagagcattctgaaactgaaggccttcagaactttttggagatgttccactttcattttgctgaagttcttcatcatccccaacacttttcattttcctcctttttcttatctggggcgtctgttcccagatgccggaggacccagcgactctgtagtgtagaatctgaggctgcagaccgccgggcacagggctgtgctcaggttctctcatggctacctttgtttttggtccatgtaactcagaacagtaaaatttcttatgattttcaaaattttccagtttcctatacctgtttctacaagtttcacactcaaacattgtccctcgcccttgatgagacttctttttttctatatgtgggccttgtgccagtgccttgctcctcactgacatggcttcaccagcagcatggcatccttggtggctctcatccagggactgtccagtaccaagaacatgactttcatttgctgaagagtcttctatggctgcttgtctcacaagtgtacggggatgcccactctggggcacaggagcgttaggtcccgatacaaagacatcatcatagaaagcgccaattttgtcatcaaatgactgacttcctcttagtggatgaggaggaggtattatatttgcaggtactgctgaataacctgtggtcggcatggaattacttcttgtgataggtaaacagtcaagtgaaggtacagacagaagaaacacttgctttgatttttcagtaggggtgaaaggtgacttcggtatatcagagcttgaacttgttctccgtcccactggttttaaatcaaactggaaagaatctttaaatatgtatgatttgggggaatcaatgcttcctcgtcttgacagtgaggttctccgcggcttcacactatccagttgcttgtcatctaccaaagcttcattgtctgagataagcttcgatatccgctcctcaagtgtttttgtggccaaaggtgggcgcatctgacctggtaaaagcaatgccttttcccctgtgggcaaagcagagggtgttgacgtggtgacaagagctgcagagggtccgttactccttccagagtcttgttctgtgctgggtaaccttctggcaaagggagttggtggactcactgtttgatcggcactttcagaacgtgaaaagtaaccagaatccgtacttcctaaacttcgaggactcaggagctttccttgctgctcttgggagtaatcggtagcctgctgcctttgtagctgggcgtgtaccgttcctacgtgagagtcttgctttccttccagtggattcatgtcgcctttctggtgggaattctcattagtctccaacctggagactccaccctgggacatgttggctgaaagtggctgtacgtttgtcacctgaaggtccttctgcttttgtgcactagaaagttcaggcttgggatccatggcctttggactgtcagttcttaagggggacacagtgacatggtggaccacaactttcggtaactctgtcacagcttgtgattctgcagatctgtcctgtagcaaaaagtcacctatcacattttctggactgcttggagtgaagcttgattttagtaaagtttcagcatttgacatcctctttattatgtgcacaggctgcagctccatggcgcccaggtcatgctgtctctcatcagtggcgccttcctcctcgctctccccactgtcttctacgtctgaatgaatactaagtgctttgggggactcgtgggacaagaacaagccaccagcatctggttgcaagacaagacccagtttgatagtatgtgcgtgggatttcttgtgcttatacagattacttttagtcttaaatgaaaatccacaagtcacacagggatagggtcgctctccagtgtgggagcggatatgctttaaaagcacactaggctttgcacatgctctattgcaatactcacaaatatattttccttgtttttttggcttctgatctttcagaagaagattgcacatttgctctacgctttgattaacaacagaggcaacatgagttgaattatagattggcatggggggcgactgtgtagaattagccggacttattgacaaaggtgaagcagaatccatttgctggttttgaggagtaacctgagatctactggaaggtgaagttaggcctacagatgatgtcactgctatattataaacctgttcaagtttggcattctcttgattttgcagatttgtcagtgatcctgtgaaacctgaacaccccggaagctgttgattatgttggttggatttgggaacaaagtgttcatgttgatgatacaaatgagaagctgactgcattgccccttgctcattcttctgagcagcagacatatggactgtgtatgaggtacaagaagactgtgattcagcaaccaattcctgtgaagtctgatttggggcatccattgaactgttttttaatttgggaggggaacgtgcagttttatttggcctcagtttttctgtcttaattgcacaaggtgagcccttttgtgacaaggtgctcagttctggctccattgctttcagtaagacatcgaatgcagtgtttgtataggagggggacgtagtgccacaatgagaagagatgcattcgctattgtcagtcctggttttacttgacaaggaacttgagtcacattgttcatcgaggtcactgaatttggcaggatcagcgccttcggatctccatctacgcagttcagatggttgctgcagaaacaagggcttctttggggagacagattcttcagattttgaggcttcagcaattattccaggtgtttctccattttgtttggtaaactgcttcccattttttacaggaatataattctgtttcttgtgagactccgaagcactatgaagaacggcgaaagatgactcttctgtattttgtttatgttttgcctgaagaggatttctcagtggggattttggtatttttttcaggtgattctcagctacgatctttttgcgtttcacacctttaagggattccgaagttcctttaacaccagcctgtaagatttctttttttgaaacttctgccccattaagttctttttgtgcttcttcaattttgtctcttagatttctgggatgaatttgtttagttcgaggcatcttctttgactcagggccttctttttcttcttaaaaactgcagataaagcaagccaccaaaaggcagctccataaactcaacatacatcaattaatccatgtgctgctcggctcgcgcgcggcgagggcgcccagaagtgccaagggtctcccgcacgcagccatcccctctgcaaggtcggcggttgcac

SEQ ID NO: 9725 - RNA, 5538 nt, Homo sapiens
  source 1..5538: mol_type = other RNA
atgcacctgggcaaggattctgatagagaagaattttggctcatctctgaaaaaacattttcacatagaaattccttctctgggtttggcaaagcattctgatgacctttttgtaatgttggcacagaattttgttcttcactgattggcactacactatgattagtctggcaaattggctgattgggcagatcttgggtcactagtatttgtggcagggatgtgagtgtagcaaaacagtaagcaggaacactactctgcaggcgtatgggcagcatgaatgatgatggcaccttctgcacctgacttccaaggggcctgagctctggtggtagcagaggatgcgaattagacatgctgtcaattaatttggttggtaatgttgctgatgtcacacaatgatctgttccaactggatctgaaataacttgatttggcaaagaatgcacaggattagaagagcaagatgggcctgaagtgaaaacctgacaatgcaattggtatttgggagcaaagcaatcctcacttttagaagacccagataaaacagaatttttatctggcttgctaccctgcgtagacacttgcagagatagctgtgtgctctggtggctaggcggtgcatggatttgatttaacaaattgatatcacagagctgttgaacaggaaaaacgttggtagagctggagtttgatgtttctgcctgcagatccttaacctgagtctgagagtgcaaagtatttgcagaaaactcagctaaagatgtactagtgagctgaggcccctgatatggcactgcattcacactgggaagagcagtattttggaaagatgttgggtgtacaggagacagatgactatctggggctatgtttaaagatatttgccgtaccagtgggcctctccttctttctaagagaggcacatgcccagtcactcccactcgagaaggtgaagatggaggctgcaattcagtaagtggtgttgtctggggtggggtgatgcttccacaatcgaatgatttgcttctgagatcagagacctccattgacgtttgcgtgcaattaatctgttctgatgcagtacgcctcatttcccggtgacatccaggaacattcagagtattcaagccagctggaatcataagaaactcggctttatttagaaaatcgattttgggggaagcctccgttttagaaacgtcctctatgtctaaagaggctgagaaacttgaagtgtgagataaactgctctccctacttagactcctggagagagtggaatcaaagctcgattctgttgaggaatgttctatctcagccagacggagccttttctttttgggtggcagtttctctgttggcaattttgacaaggtttcactacgctggggccaactgaacttctctgacttttcttgatcatggcattgagcttccaggtctcgatctggttcttctgtgaccaaaatctctggaacttggatgttgtgctgccggacaagtcttgagggctgtcctaacacatgtcgttcacttggactctttctggagctttcctgaagttctcctctgagagcgtctgatagtgcaagctggtgaggatgagacccgtcccgagaagggtgactttcctcttgggagattcctatcacttttagagacccggacttccccgttctattcagctcctggaaagaaactggggaggctctttcaaaaggctcaggcttgtcaaatgagttgggcctgctcagggagttggtgtgctggatgacagagattccagttccgtgtctctgcagttctatcttgtcctgggctgctgaacttatctgttgttccatgatggtcgacagcttgggatccatggtctgctcagggcccctggcaacaaggtgaatatgggagttttgcaactgtatatttttatgctgctggtcacttcttatggtaacattatgtttaggcaaactgggattacagcccagagcattctgaaactgaaggccttcagaactttttggagatgttccactttcattttgctgaagttcttcatcatccccaacacttttcattttcctcctttttcttatctggggcgtctgttcccagatgccggaggacccagcgactctgtagtgtagaatctgaggctgcagaccgccgggcacagggctgtgctcaggttctctcatggctacctttgtttttggtccatgtaactcagaacagtaaaatttcttatgattttcaaaattttccagtttcctatacctgtttctacaagtttcacactcaaacattgtccctcgcccttgatgagacttctttttttctatatgtgggccttgtgccagtgccttgctcctcactgacatggcttcaccagcagcatggcatccttggtggctctcatccagggactgtccagtaccaagaacatgactttcatttgctgaagagtcttctatggctgcttgtctcacaagtgtacggggatgcccactctggggcacaggagcgttaggtcccgatacaaagacatcatcatagaaagcgccaattttgtcatcaaatgactgacttcctcttagtggatgaggaggaggtattatatttgcaggtactgctgaataacctgtggtcggcatggaattacttcttgtgataggtaaacagtcaagtgaaggtacagacagaagaaacacttgctttgatttttcagtaggggtgaaaggtgacttcggtatatcagagcttgaacttgttctccgtcccactggttttaaatcaaactggaaagaatctttaaatatgtatgatttgggggaatcaatgcttcctcgtcttgacagtgaggttctccgcggcttcacactatccagttgcttgtcatctaccaaagcttcattgtctgagataagcttcgatatccgctcctcaagtgtttttgtggccaaaggtgggcgcatctgacctggtaaaagcaatgccttttcccctgtgggcaaagcagagggtgttgacgtggtgacaagagctgcagagggtccgttactccttccagagtcttgttctgtgctgggtaaccttctggcaaagggagttggtggactcactgtttgatcggcactttcagaacgtgaaaagtaaccagaatccgtacttcctaaacttcgaggactcaggagctttccttgctgctcttgggagtaatcggtagcctgctgcctttgtagctgggcgtgtaccgttcctacgtgagagtcttgctttccttccagtggattcatgtcgcctttctggtgggaattctcattagtctccaacctggagactccaccctgggacatgttggctgaaagtggctgtacgtttgtcacctgaaggtccttctgcttttgtgcactagaaagttcaggcttgggatccatggcctttggactgtcagttcttaagggggacacagtgacatggtggaccacaactttcggtaactctgtcacagcttgtgattctgcagatctgtcctgtagcaaaaagtcacctatcacattttctggactgcttggagtgaagcttgattttagtaaagtttcagcatttgacatcctctttattatgtgcacaggctgcagctccatggcgcccaggtcatgctgtctctcatcagtggcgccttcctcctcgctctccccactgtcttctacgtctgaatgaatactaagtgctttgggggactcgtgggacaagaacaagccaccagcatctggttgcaagacaagacccagtttgatagtatgtgcgtgggatttcttgtgcttatacagattacttttagtcttaaatgaaaatccacaagtcacacagggatagggtcgctctccagtgtgggagcggatatgctttaaaagcacactaggctttgcacatgctctattgcaatactcacaaatatattttccttgtttttttggcttctgatctttcagaagaagattgcacatttgctctacgctttgattaacaacagaggcaacatgagttgaattatagattggcatggggggcgactgtgtagaattagccggacttattgacaaaggtgaagcagaatccatttgctggttttgaggagtaacctgagatctactggaaggtgaagttaggcctacagatgatgtcactgctatattataaacctgttcaagtttggcattctcttgattttgcagatttgtcagtgatcctgtgaaacctgaacaccccggaagctgttgattatgttggttggatttgggaacaaagtgttcatgttgatgatacaaatgagaagctgactgcattgccccttgctcattcttctgagcagcagacatatggactgtgtatgaggtacaagaagactgtgattcagcaaccaattcctgtgaagtctgatttggggcatccattgaactgttttttaatttgggaggggaacgtgcagttttatttggcctcagtttttctgtcttaattgcacaaggtgagcccttttgtgacaaggtgctcagttctggctccattgctttcagtaagacatcgaatgcagtgtttgtataggagggggacgtagtgccacaatgagaagagatgcattcgctattgtcagtcctggttttacttgacaaggaacttgagtcacattgttcatcgaggtcactgaatttggcaggatcagcgccttcggatctccatctacgcagttcagatggttgctgcagaaacaagggcttctttggggagacagattcttcagattttgaggcttcagcaattattccaggtgtttctccattttgtttggtaaactgcttcccattttttacaggaatataattctgtttcttgtgagactccgaagcactatgaagaacggcgaaagatgactcttctgtattttgtttatgttttgcctgaagaggatttctcagtggggattttggtatttttttcaggtgattctcagctacgatctttttgcgtttcacacctttaagggattccgaagttcctttaacaccagcctgtaagatttctttttttgaaacttctgccccattaagttctttttgtgcttcttcaattttgtctcttagatttctgggatgaatttgtttagttcgaggcatcttctttgactcagggccttctttttcttcttaaaaactgcagataaagcaagccaccaaaaggcagctccataaactcaacatacatcaattaatccatgtgctgctgccaggacgcccggcggagccgctgccgctgcagccggccctggagctgcgctgctgatggcggcggccgcggctcgggatctccgcgacccccgcgcggcggcggcggcggcgcctgggatccctccttcacttgacaaccccaaacacaaacataacctcctccggcggccgccgctccccggtcccccgctccgtccgccaccctgccgccgcccagcagccgccacgctgaaggccggcgactggc

SEQ ID NO: 9726 - RNA, 72 nt, Homo sapiens
  source 1..72: mol_type = other RNA
atgcctcccccggccccgcagcgccccgtccgcggacgagcagggaagcccgggaggcgccgggcgggcaac

SEQ ID NO: 9727 - RNA, 75 nt, Homo sapiens
  source 1..75: mol_type = other RNA
atgcctcccccggccccgcagcgccccgtccgcggacgagcagggaagcccgggaggcgccgggcgggcaacgct

SEQ ID NO: 9728 - RNA, 669 nt, Homo sapiens
  source 1..669: mol_type = other RNA
atgcctcccccggccccgcagcgccccgtccgcggacgagcagggaagcccgggaggcgccgggcgggcaacgctggtcctttcaaaggcacccgctttcctaagcgttagccgtctgaaaatcatccgcatttttcatgtaaaccacatctgtgtttctttgttggtggtatttttctttgacggaacggacacgttttactgaaatgtatttattcaaaaagctcacacgactcccatataggagaaatcagggtaaggaacgtaaggcaacgagacggccaccgccgccgagctctgggttccgccctctcttcctcccctcggggcgggcctcacctcaggtcggcggcgaagaactcgaagtagtcgtgtgctggcagcgggcgcagctgctcctccagctgctccttggtgaggcccggaggcaggcggcggatgaccaccttgctcagggccgtcctcttctcctcgcgaggtttgcccgcaccgcccccgcaaccggaggacgaagttggcggcgtctcagcctcctgctgctgcgagtcgcggtggaactgcacttctagggccgacagcttctccctcccgctcgggccccgcgcggcaacggccgcccgaaggcctccggccccctccttttccgagcgcatgccgcactctccgccg
